European Patent Application EP 4 520 821 A1 - sequence listing, part 8

SEQ ID NO: 13704 - RNA, 11308 nt, Homo sapiens
  source 1..11308: mol_type = other RNA
gctgggattacaggcatgagccaccatgcccagctaatttttgtatttttagtagagacagggtttcaccatgttggccaggctggtcttgaactcctgagctcgggtgatctgcctgcttcagcctcccaaagtgctgggattacaagtgtgagccaccctgcacggcccctttctttctggcttcctcctcccttcttccttttctttcatttttaaaacatttttttaaaattattatttttaaatttttttttttgagatggagtctagctctgtcgcccaggctggagtgcagtggcatgatcttggctcactgcaatctctgcctcccgggttcaagcaattctcctgcttcagcctcccgagtagctgggattacaggtgtccaccaccacacccagctaatttttgtatttttagtagacggggtttcactgtgttggccaggctggtcttgaactcctaaccttgtgatccttggcctcccaaagtgctgggattacaaacgtgagctactgcgcctggcctattattattatttttgagacagagttttgctcttgttgcctgggtgggagtacaatggcgtgatcttggctcactgcaacatctgcctctcggtttcaagcgattctcctgcctcagcctctcaagtagctgggattacaggcgtgagccaccacacccggctaatttttgtatttttagtacagacggattttcaccatgttggccaagctggcctcgaactcctgacctcaggtgatctgcctgcctcagcctcccagagtgctgggattacaggcgtgagccaccgcgcccggcctaaaattatttttttagagacagggtctgactctgatgtccaggctggagtgcagtggcgctattatagctcactgctgtcttaaactcttgtgctcaagtaatcctcctgcctcagcctcccgagtaggtgggaccacaggcatgtgccaccatgcccagctcatatttttaattattgaaaaaaaaaaaacccaattttaaaaaccacacacagactcaaatgggcacagcaccaaattatgacacattagaatccttcctatgtgctcagagaacagggtttgtgctgagcttgagataaggcttctcttgctgtccctgtcaatcaaagagactgcaaggtgggcttcagacacagtgctagcatttgtaaacaattatctgtgagaatcagcggtcactttgtcctgtgctaccaaaatcaaacactgaaagaaaatggacattgagaccaacataagactacaactaccatcccagcccccagttcaaacatttgtgttcattgctcttcgccctgatggactgtatgctaagaaagaatttgcacttgcaaaatacatttttgctaactagatgctcattttatctttttaaaaatatgtatttcagttgcacatgaaatgtactttgaaagaatgagctccaaagttctggggggctgagacaggcgggctgagtgaaatgatgaagaaacagtggctttcagtgcgggccaagagagtagtgagcaatggtcagttattgagctgtggagtgccttcaacaagggtttttagacacatccatctggtgcctcatcccagaacctcacaggcctagggacctgaaatgctccccatgacaaggcaaacttcatatcctcacatgctgagacagactcaactttcagtctggaactgggctgggtgtctgtcagtccacgccacccatatccggagtacatcagagtctgggttcagtggcagccactttcgctgccctctcctgccccacacctagcgctctgcctggcccctttgctgtgggcgtgaaaatctggcacccgggccgacagggagagagctcagtctgcgtctgctgctttctgtttgattcatcactttccccttcaccctggagcccacgttggctgtggggcacctaactggctcctgaggcccctctggggggttgaggccctgggctgcatttggcctcggcagcctgctcacgcctctcctgactgggatgtcagaggactaggttcaaactccagcatggccagctgctggctgtgtgaccttgggcatgttaagcctcagtcccttcatccatacagtgggccaaggaagggatccctgatgtgccaacagatggatttatgaccacgtgtgtgcagcacctggcactagtttacacactgcagatgcccggtactgttgtcgccagcactcaggtctaggagagtggtcttcacaactctacctcaagggttgcctttggactgtgtccccacatggtcacatttgcatctccagacgccccaatgctgcttctcggatattctgaaggcatcctacactgtcaagctccccgactgttccccccagcaccccagtctccaactcagggtggccccatttcccccaggtcccaatcagatccctgggcccactgtggtcctggccatctcacatccaaaccctcagcaatggttgtgagtcagttctgttccagaatatctgatgccactgctacagaccccagccacctccagaccctggacaagttgcagcctcctgccccagcccctttttcctggcagccagaaagagcagcctcaatgcttctctaaccctgtaactcagctcaaaaagctctttaggcccctggtccccagaaatgcattcagagctcagccaaggggacctctcggcaccacctcacccctacatatccctacccgcatgtctgcagaactccaggcttttgtccagactgtccctactgcctggtatattcctgtcctatccgcccctcctcaagcctggtgtgatgactaaggcctccagctccaggtcactcagcctatgccagaatcacagctcagccagcctatgagcaagtttcttagccccagtttgtttcttcgtcagtataacgagagggttcacagcctccatctctgaggatgtcatgaaggttgagtaagataatcctggaagtacttggcgcaggatgcaccatattctataggaccctccacttggtatcatctccctggtgcctgacacaaagtaggtcttgagagactgaggccctggccctatacctcaggagatgcacccaggagcagctgcaggtcttctagaaagccctctagggacagccctggaaacccttgctcctgctccaagggtccacaagcccaggtaacttctgcgctaagctctgcaggggacagcccaggacctagttatgctggcctcagcgtctctgatagtcaaatggacaccaatggcagcctcatcctcccttcctgtccagctatgcaacctgacctgcaactgcaccctgctgagccttggtgtcctcaactttgtaatgtggggacaactaaaaaccccatgtgccagccctggcaacatagcaagaccccgtttctaaaaaaaaaaaaaaattaaaaattagccaggcagggttgttcacacctgtagtcctagtttgctttgcttggtcacgtagctcagcctcacactgacttccaggaacagcagagggacttggacgcctctccaggcaggcaggcctgttcctggaaagccaggtggggtggggggtcttcaggtggcaaaggaaggactggcagctgtgagccagagaagagacctggctcgtgccccagccctgctcctgtcctgctaagcctcagtttcctcatctgtaccacagggatctctgtgagcgcttcaggcaccaacaatctgctccctgggctcagtaggggatatctgatcccaccatttccccagccacatgccccagaagagggccgcagacctagtacaagagggagcaataaggtgacatcctctgctctgagaggtagagtgtttggggaagaccccagcccctgggaagggggccacttagccaggcctgcctgccacggggcatggctactctaagctgtctcaccctccccctttaggcatagctggggcaggtggaggtcagcccagttcagggctttccatgaagctgaggtaggcttccctgcctttcccactttgtgagctgtaaaattagcctttcctgaccattttcctgcaggactgctgtatgtgtgagaggtagtctttggaagaaaaggggcctctagaatttgaagcttctgatttctggttatgaggccaaagatcccaaaggtccttccagacacctcaggagggccctggggggcagaggctgggggctgtacagccaattacctcagaggggaaggcacccactcattccgcaagcgggggaaatcctgctctcctcccacagctaccagagcttcagatgggactcagatctgtctgcacacccagggctacagttggcctaatgtgactcttacctgcccataaacctggcccagagggctttatgggccagaatccctgggtttagtagctacatggacagccatatgagcaccacctaattgacttaattaactaaccccaggcctttggaagcaataggagatgagagcatcatactgggagtcaggagtcaagtgctgtgttacttcaagtaagccccatccctctctgggaaaaaagatcagggattgaatataagtcttgccatgatccaccccttccagtataaacaggccctcctggcttcatccaaagcgtatccaggtgatttggggccaagctgacccttgaacccaggtgtccatgctctctgtcccccagcttctcagctctgaaacccagcatgaggcccatgtctggcctcccagtagctctccatgtggctcctgggttaggactggcttcaggagccccaagccttggctgggtgggatggtgtctccagagtcctttagtacccctggaaagggaggtcctagtcccagcttggacagggacagggctgagggcaccagttggccaattcagttttaggaaccaggaggttgagaaccccagggatagccccactccaccataggaacagaatggtgacacagctctgctcaggcctatggcttacatggaggggccaggcccattagctcaaagtcaggggctgctgtgctcatttcacagatgcagtacctgcaacccagagagtacagggcccctgctcatcctcacacacccaaggggtcctgggccagtcacataactccacaggagagcaggaacaggcttggtcccagtctctgaggtcctctctggacccagtctctggagatgggccatggaggccagccttgcactttctccccacatcccagtcccattcctcacccactcccttctgggacccatgctggtcagtctttcagtcttctcactctgggaaagggccacctctctccaaatatgagtaaaaaaagggggggcctgggcagtttaggtctgaaggttgaggaagagttcccctggccacatcacctatcagaagagaggtggttaaggcaatttatcatgactctcaaaattcttccagcctctgcccatttccacgttgcaattccaaagccacttcaatcagtaggcgtgtgttacagcagcactctaatttgggcaccacaatctatattcgtttcccgtggctgctgtaacaaattatcacacatgtgttttcacacatgtgaaaacaacacaaatttatgatcttactgttctggaggtcagcaatctgaaatcagtttcacagggcttaaaatcaaggtattggcaggactgcattcttcttgaggccccagaggagaagaggctgtctgcattcctcggctcatggctcttcctccagcaattgcatcactctgacctctgcttccattgttacatacattttcttccgtcactctgacactcctgcctcctttacagaggcccttgtgattatactcagtttacctgaaaaatccaggatactccttccatctcaagatccttaatcacatctgcaaagtccattttgctatgtgaaggtaatatagtcacatgttaaggtttaggtgattaagacactgccattttggggggtcactgttcagcctaccagagcaggggtagagttgctttgacagtcccaaatccagttcagggggcttgtccagggcagaaggtcatgaggaggagatcaggtcactgtcctagccaggactctggctgggggctggctgaagccaagagctccaggaaacctggcgcctgctcctactgccgccaaggacagcctgttctcctggtgtggctgttgcgcagggatcaggtgcacttgagtcttcgaagtggccattgctcaacttgaatggctgcctgggtcgggcagaaggccaggtcctcatggcttcccatccctaatgaccggaatacatgggctgccaggtcagatgtgggccacatgggaagtcccagctctattctagaaaatgcatgtaccatcagcttactgatagacatttactgaacttgggtatgccagatccacagggggccccagagatgagggggataagaaggtttctgaaggcatggtacagaaggtgccagcagaggtatgggctaggggaggcagggagagcacagagcaggcatcctaaaggaggcagcatttgtgttggagcttgaagaagtggattgtttgcaccgcctgggcaaagggaaggtgtgtgttcagggcatcgagagtactgcacaaaggctgaagcccagggcagtagagaagagaatccactaagaaggagccaatgaagaaaaaaaagagaaaagaatcgaaggtggatagggaaagacatgctgtcccgcagaggttaaaggggttctcacctcaagccagcagttctcaaaccttgtcagcagtggagccctttgttctgatgacagcctactcagagcactgatggggccttgggaggggcccccagggcttttcccacagttgtcctcccccacctcttcagaactggattccataggacacaagagaacacacttaagtcatggggagccagctaagtgtttggggcaaggattgggagcagccaatagcccagggtccaggtgggggtaaaggagcaaaaaagagtattttttgcatttagggggttcggggcctatttcaataaggcagctgtatgagacccatggagaaacccactgacaactgggaaaagcatccaactgtgagacaaggcctcagtttccccaactatcagaagaggagatagaattactctcccagagtacatcaaacagggactcctacactcctgtctatgctctgggctctggctgaaggaggctgcacgggcagtgggcacatctctcaagacctcaggggcttgcacagcctggactccatcagctccatgtcctcctcccattctgcctgcaagtgctccttgacatatgctggtggtggtggggaggctgttcgagtctctggctttggcctcaggagcaagggaggggatagggcaggtgggcctggctttccctgagctagagccactggctgccctggcctgggcctcaaggcactggggccatagtgaggagaggctgaggggagatgtaggctgccaggctaccagcctgctggctccatctctagacaacagtgaggagtcaagagcccaagactgaaactcctgccttcccttctttccagactgccttgtatccctgcctgccttatgttggtcccatgcatcagatggacgcctgagggcactgggtccttcctccctgtgtctgccctccgaggaaggcaaggaaaaatgccacaatgtgccaagccaggcacatcccatgggctcctcacatgcatcctataaaataaagcattaagtcccatttctcagccttagaagccaaggctgagtgaggtgaagtcatctgcccaaggtcacatcctcgtgaggggcagattctgggattgaaatccaggctggtgtggctccaacatctgggctcaacgtccagggcccaatcaagccagtggctgcaggcttgaggccccgcctgccagtcctcttggcttggaccttttcctcagcagagtcaagctgcacatttttctgggcagaaagttgtgcccgaggccggctcctgcttgtggccccagctgccccgacagtgtcactctccaacactgcactctcttctggtgcaacatccacaagctcgccaaggcccttcctcaggaatgggcctgaggccaggagggagagaccatcagggaagccaggactggctgaggtgtaggggggcgacagactgctccgaggtcagggcagctaccctgagatgctgctgaagacagcaagagccaaagggcacaaggagaaagacagaaagggcaatactggtgaggaccttagcaggcaaaggtctgtgagcatgggggactaaggaagtggggagccttgccctggttgtgcacccccttcgccctccccacccaggttccttctggagcagcctccttaaaggaagccaggggcagctcagagtccatgcagctggggctgggcacagggcaggacactggggcactgggagctgcagtgtgacctctaccaaatgtgtcctccagccatagtgcagggcaacacttaggctgggtatgactccagcaatataggctccccaaagggagggatctaacttactgtctccacttggtcactgtcatgtgacctcaggcagtacataccttctcttgctctccatgcctggcgaatggacattcagatgccagcatgcacattccacttgactaagagtaaagaggttgccagttggcgttggccctggactcagaagagccagcttctcatagggaaaggagttgcccaaggtcccactgcaggacacagccctggaactcagctctcccagctgcagcagaggatgctgcctattggaccatactgcccatcagaccatactgccaggccctgggaagtgccagggtggcagggggcagtctagtggaatgagacagcctggtttgccatgtttcttaggacccaccctgatgtaggctcacatcaccagcactcaccaacctagagatttcctgtcgctgttgacaggaaggctggatctgcaggcctcctggtggccatgagtctgcacagaccagagctggggtggaggccacaaccctgtgcccagtatctcagcttctcactctccccagccccaaccagggacacatgggttatttgaaaccccagggggtcaactcgggagggatgttttagctaaaagctatggggataaaaaggaaacacccctcactggctcaagccttcagttaaatgaacgtggatgtgcgacccaggaactgtgcagcaaagacctccagaccctcccctccagaaagcaggcagtcatccttgagccaaaacgcagatgagcttcctgtgctcgagccaggcttggccagggaattgtgtacgcatgcacccagggcagtggaggactaatcaatccctgggagtgagctgctctatgccaggacccatggtatccaaggccaggagtgaggactcacgtgccttcctccacactgcacccccacaccactaccaagcaggggactgacggccagccctgctggggcagaaggaaacccttgccccagtgctacctgggagtaagggggtcaggggacctgcaagtcatggacaaaacattaggtcaccatttgttagtctctcaatactttactggccatatcccccgatacccccacagcaatttcaccaacacagagcaactgccctcagccactctgatgtgatggagccaatccaggtgtcctagaaatatcctagaaatgcagagcatggggaaatcacagaaccctgggaaatgccataagaacctgggctctggaaagtgccatccacctcccctctggtcaggctggcggcactgacaaggcatccacagggcagccatgctatggcccagacctccggatatgcaggaaccggggcctcccacagaagtccctgcgcacagccacaagattaaggtacaggtcaggccggctctgaagccagctgctgacaagctccgggtgccttgggtccacttctaagaagatactaccagagtctttcaggagccggggtgccaaggccagaatgtgggtaatgatgtccatgccctcctccccaccatccagggccgcggggtcttcatagctgcggatctcaggggccagctgctccatgtcctggtggaagacgtagggagggttgctgacaatcaggtccatggggccccagggcaggtgtgtccagctcctttctgaggtcatgtcgaggtggatgatccaaatcctgtcctgcaaccgaagcctctgagcattctcatgggtcagagagatagcagcttcccgcttatccacagcaatgactcggctctgggggagctggctcagcaggctgagggagatggctcctgatccgcagcccacctccagaatgagggggctgcctggggatcccacagcatgggacctctgggccacctcttccagcacccactcaaccagttcctctgtttctggccgaggaataaacactgggggcaccatccttaggctgagcccctggaagtcccactctccaaggatgtactgcaccggcatcctgcagagggggcagctgggtggtcatcagggacagagctctgcaatcgacggctactcagctcccggatacactgtagttgctgagaggtcaagggctgggtccaaagtgccggcctcaggctctgaaatgttttggctccaaggacatgagccacgatgtactcactggattcccgggcctcagggatacccctcttctcaaagaccccagtccagtggctgaccagttctatggcactggataacccagccagaggtggttggggttgccatgagctgaaggcccagccccgggtacttcccctcctccctgggccagacaggagggcccacagcattcggccccaaagctccatgtctcagggaaaggttctccagagtgcttccaggttcccaagtctgctttatgatgtcagctgctgaggtgagtgctgagagtggcccctggacccagctgggtggagatggagaggtcacaagctctggtgccccaaaatggctctggtcctcagatatagttggttgccaccctgcctgaaaggctgccccacccacccaccagccggagaagctgccccgaact

SEQ ID NO: 13705 - RNA, 9636 nt, Homo sapiens
  source 1..9636: mol_type = other RNA
gctgggattacaggcatgagccaccatgcccagctaatttttgtatttttagtagagacagggtttcaccatgttggccaggctggtcttgaactcctgagctcgggtgatctgcctgcttcagcctcccaaagtgctgggattacaagtgtgagccaccctgcacggcccctttctttctggcttcctcctcccttcttccttttctttcatttttaaaacatttttttaaaattattatttttaaatttttttttttgagatggagtctagctctgtcgcccaggctggagtgcagtggcatgatcttggctcactgcaatctctgcctcccgggttcaagcaattctcctgcttcagcctcccgagtagctgggattacaggtgtccaccaccacacccagctaatttttgtatttttagtagacggggtttcactgtgttggccaggctggtcttgaactcctaaccttgtgatccttggcctcccaaagtgctgggattacaaacgtgagctactgcgcctggcctattattattatttttgagacagagttttgctcttgttgcctgggtgggagtacaatggcgtgatcttggctcactgcaacatctgcctctcggtttcaagcgattctcctgcctcagcctctcaagtagctgggattacaggcgtgagccaccacacccggctaatttttgtatttttagtacagacggattttcaccatgttggccaagctggcctcgaactcctgacctcaggtgatctgcctgcctcagcctcccagagtgctgggattacaggcgtgagccaccgcgcccggcctaaaattatttttttagagacagggtctgactctgatgtccaggctggagtgcagtggcgctattatagctcactgctgtcttaaactcttgtgctcaagtaatcctcctgcctcagcctcccgagtaggtgggaccacaggcatgtgccaccatgcccagctcatatttttaattattgaaaaaaaaaaaacccaattttaaaaaccacacacagactcaaatgggcacagcaccaaattatgacacattagaatccttcctatgtgctcagagaacagggtttgtgctgagcttgagataaggcttctcttgctgtccctgtcaatcaaagagactgcaaggtgggcttcagacacagtgctagcatttgtaaacaattatctgtgagaatcagcggtcactttgtcctgtgctaccaaaatcaaacactgaaagaaaatggacattgagaccaacataagactacaactaccatcccagcccccagttcaaacatttgtgttcattgctcttcgccctgatggactgtatgctaagaaagaatttgcacttgcaaaatacatttttgctaactagatgctcattttatctttttaaaaatatgtatttcagttgcacatgaaatgtactttgaaagaatgagctccaaagttctggggggctgagacaggcgggctgagtgaaatgatgaagaaacagtggctttcagtgcgggccaagagagtagtgagcaatggtcagttattgagctgtggagtgccttcaacaagggtttttagacacatccatctggtgcctcatcccagaacctcacaggcctagggacctgaaatgctccccatgacaaggcaaacttcatatcctcacatgctgagacagactcaactttcagtctggaactgggctgggtgtctgtcagtccacgccacccatatccggagtacatcagagtctgggttcagtggcagccactttcgctgccctctcctgccccacacctagcgctctgcctggcccctttgctgtgggcgtgaaaatctggcacccgggccgacagggagagagctcagtctgcgtctgctgctttctgtttgattcatcactttccccttcaccctggagcccacgttggctgtggggcacctaactggctcctgaggcccctctggggggttgaggccctgggctgcatttggcctcggcagcctgctcacgcctctcctgactgggatgtcagaggactaggttcaaactccagcatggccagctgctggctgtgtgaccttgggcatgttaagcctcagtcccttcatccatacagtgggccaaggaagggatccctgatgtgccaacagatggatttatgaccacgtgtgtgcagcacctggcactagtttacacactgcagatgcccggtactgttgtcgccagcactcaggtctaggagagtggtcttcacaactctacctcaagggttgcctttggactgtgtccccacatggtcacatttgcatctccagacgccccaatgctgcttctcggatattctgaaggcatcctacactgtcaagctccccgactgttccccccagcaccccagtctccaactcagggtggccccatttcccccaggtcccaatcagatccctgggcccactgtggtcctggccatctcacatccaaaccctcagcaatggttgtgagtcagttctgttccagaatatctgatgccactgctacagaccccagccacctccagaccctggacaagttgcagcctcctgccccagcccctttttcctggcagccagaaagagcagcctcaatgcttctctaaccctgtaactcagctcaaaaagctctttaggcccctggtccccagaaatgcattcagagctcagccaaggggacctctcggcaccacctcacccctacatatccctacccgcatgtctgcagaactccaggcttttgtccagactgtccctactgcctggtatattcctgtcctatccgcccctcctcaagcctggtgtgatgactaaggcctccagctccaggtcactcagcctatgccagaatcacagctcagccagcctatgagcaagtttcttagccccagtttgtttcttcgtcagtataacgagagggttcacagcctccatctctgaggatgtcatgaaggttgagtaagataatcctggaagtacttggcgcaggatgcaccatattctataggaccctccacttggtatcatctccctggtgcctgacacaaagtaggtcttgagagactgaggccctggccctatacctcaggagatgcacccaggagcagctgcaggtcttctagaaagccctctagggacagccctggaaacccttgctcctgctccaagggtccacaagcccaggtaacttctgcgctaagctctgcaggggacagcccaggacctagttatgctggcctcagcgtctctgatagtcaaatggacaccaatggcagcctcatcctcccttcctgtccagctatgcaacctgacctgcaactgcaccctgctgagccttggtgtcctcaactttgtaatgtggggacaactaaaaaccccatgtgccagccctggcaacatagcaagaccccgtttctaaaaaaaaaaaaaaattaaaaattagccaggcagggttgttcacacctgtagtcctagtttgctttgcttggtcacgtagctcagcctcacactgacttccaggaacagcagagggacttggacgcctctccaggcaggcaggcctgttcctggaaagccaggtggggtggggggtcttcaggtggcaaaggaaggactggcagctgtgagccagagaagagacctggctcgtgccccagccctgctcctgtcctgctaagcctcagtttcctcatctgtaccacagggatctctgtgagcgcttcaggcaccaacaatctgctccctgggctcagtaggggatatctgatcccaccatttccccagccacatgccccagaagagggccgcagacctagtacaagagggagcaataaggtgacatcctctgctctgagaggtagagtgtttggggaagaccccagcccctgggaagggggccacttagccaggcctgcctgccacggggcatggctactctaagctgtctcaccctccccctttaggcatagctggggcaggtggaggtcagcccagttcagggctttccatgaagctgaggtaggcttccctgcctttcccactttgtgagctgtaaaattagcctttcctgaccattttcctgcaggactgctgtatgtgtgagaggtagtctttggaagaaaaggggcctctagaatttgaagcttctgatttctggttatgaggccaaagatcccaaaggtccttccagacacctcaggagggccctggggggcagaggctgggggctgtacagccaattacctcagaggggaaggcacccactcattccgcaagcgggggaaatcctgctctcctcccacagctaccagagcttcagatgggactcagatctgtctgcacacccagggctacagttggcctaatgtgactcttacctgcccataaacctggcccagagggctttatgggccagaatccctgggtttagtagctacatggacagccatatgagcaccacctaattgacttaattaactaaccccaggcctttggaagcaataggagatgagagcatcatactgggagtcaggagtcaagtgctgtgttacttcaagtaagccccatccctctctgggaaaaaagatcagggattgaatataagtcttgccatgatccaccccttccagtataaacaggccctcctggcttcatccaaagcgtatccaggtgatttggggccaagctgacccttgaacccaggtgtccatgctctctgtcccccagcttctcagctctgaaacccagcatgaggcccatgtctggcctcccagtagctctccatgtggctcctgggttaggactggcttcaggagccccaagccttggctgggtgggatggtgtctccagagtcctttagtacccctggaaagggaggtcctagtcccagcttggacagggacagggctgagggcaccagttggccaattcagttttaggaaccaggaggttgagaaccccagggatagccccactccaccataggaacagaatggtgacacagctctgctcaggcctatggcttacatggaggggccaggcccattagctcaaagtcaggggctgctgtgctcatttcacagatgcagtacctgcaacccagagagtacagggcccctgctcatcctcacacacccaaggggtcctgggccagtcacataactccacaggagagcaggaacaggcttggtcccagtctctgaggtcctctctggacccagtctctggagatgggccatggaggccagccttgcactttctccccacatcccagtcccattcctcacccactcccttctgggacccatgctggtcagtctttcagtcttctcactctgggaaagggccacctctctccaaatatgagtaaaaaaagggggggcctgggcagtttaggtctgaaggttgaggaagagttcccctggccacatcacctatcagaagagaggtggttaaggcaatttatcatgactctcaaaattcttccagcctctgcccatttccacgttgcaattccaaagccacttcaatcagtaggcgtgtgttacagcagcactctaatttgggcaccacaatctatattcgtttcccgtggctgctgtaacaaattatcacacatgtgttttcacacatgtgaaaacaacacaaatttatgatcttactgttctggaggtcagcaatctgaaatcagtttcacagggcttaaaatcaaggtattggcaggactgcattcttcttgaggccccagaggagaagaggctgtctgcattcctcggctcatggctcttcctccagcaattgcatcactctgacctctgcttccattgttacatacattttcttccgtcactctgacactcctgcctcctttacagaggcccttgtgattatactcagtttacctgaaaaatccaggatactccttccatctcaagatccttaatcacatctgcaaagtccattttgctatgtgaaggtaatatagtcacatgttaaggtttaggtgattaagacactgccattttggggggtcactgttcagcctaccagagcaggggtagagttgctttgacagtcccaaatccagttcagggggcttgtccagggcagaaggtcatgaggaggagatcaggtcactgtcctagccaggactctggctgggggctggctgaagccaagagctccaggaaacctggcgcctgctcctactgccgccaaggacagcctgttctcctggtgtggctgttgcgcagggatcaggtgcacttgagtcttcgaagtggccattgctcaacttgaatggctgcctgggtcgggcagaaggccaggtcctcatggcttcccatccctaatgaccggaatacatgggctgccaggtcagatgtgggccacatgggaagtcccagctctattctagaaaatgcatgtaccatcagcttactgatagacatttactgaacttgggtatgccagatccacagggggccccagagatgagggggataagaaggtttctgaaggcatggtacagaaggtgccagcagaggtatgggctaggggaggcagggagagcacagagcaggcatcctaaaggaggcagcatttgtgttggagcttgaagaagtggattgtttgcaccgcctgggcaaagggaaggtgtgtgttcagggcatcgagagtactgcacaaaggctgaagcccagggcagtagagaagagaatccactaagaaggagccaatgaagaaaaaaaagagaaaagaatcgaaggtggatagggaaagacatgctgtcccgcagaggttaaaggggttctcacctcaagccagcagttctcaaaccttgtcagcagtggagccctttgttctgatgacagcctactcagagcactgatggggccttgggaggggcccccagggcttttcccacagttgtcctcccccacctcttcagaactggattccataggacacaagagaacacacttaagtcatggggagccagctaagtgtttggggcaaggattgggagcagccaatagcccagggtccaggtgggggtaaaggagcaaaaaagagtattttttgcatttagggggttcggggcctatttcaataaggcagctgtatgagacccatggagaaacccactgacaactgggaaaagcatccaactgtgagacaaggcctcagtttccccaactatcagaagaggagatagaattactctcccagagtacatcaaacagggactcctacactcctgtctatgctctgggctctggctgaaggaggctgcacgggcagtgggcacatctctcaagacctcaggggcttgcacagcctggactccatcagctccatgtcctcctcccattctgcctgcaagtgctccttgacatatgctggtggtggtggggaggctgttcgagtctctggctttggcctcaggagcaagggaggggatagggcaggtgggcctggctttccctgagctagagccactggctgccctggcctgggcctcaaggcactggggccatagtgaggagaggctgaggggagatgtaggctgccaggctaccagcctgctggctccatctctagacaacagtgaggagtcaagagcccaagactgaaactcctgccttcccttctttccagactgccttgtatccctgcctgccttatgttggtcccatgcatcagatggacgcctgagggcactgggtccttcctccctgtgtctgccctccgaggaaggcaaggaaaaatgccacaatgtgccaagccaggcacatcccatgggctcctcacatgcatcctataaaataaagcattaagtcccatttctcagccttagaagccaaggctgagtgaggtgaagtcatctgcccaaggtcacatcctcgtgaggggcagattctgggattgaaatccaggctggtgtggctccaacatctgggctcaacgtccagggcccaatcaagccagtggctgcaggcttgaggccccgcctgccagtcctcttggcttggaccttttcctcagcagagtcaagctgcacatttttctgggcagaaagttgtgcccgaggccggctcctgcttgtggccccagctgccccgacagtgtcactctccaacactgcactctcttctggtgcaacatccacaagctcgccaaggcccttcctcaggaatgggcctgaggccaggagggagagaccatcagggaagccaggactggctgaggtgtaggggggcgacagactgctccgaggtcagggcagctaccctgagatgctgcttctcttgctctccatgcctggcgaatggacattcagatgccagcatgcacattccacttgactcccacagaagtccctgcgcacagccacaagattaaggtacaggtcaggccggctctgaagccagctgctgacaagctccgggtgccttgggtccacttctaagaagatactaccagagtctttcaggagccggggtgccaaggccagaatgtgggtaatgatgtccatgccctcctccccaccatccagggccgcggggtcttcatagctgcggatctcaggggccagctgctccatgtcctggtggaagacgtagggagggttgctgacaatcaggtccatggggccccagggcaggtgtgtccagctcctttctgaggtcatgtcgaggtggatgatccaaatcctgtcctgcaaccgaagcctctgagcattctcatgggtcagagagatagcagcttcccgcttatccacagcaatgactcggctctgggggagctggctcagcaggctgagggagatggctcctgatccgcagcccacctccagaatgagggggctgcctggggatcccacagcatgggacctctgggccacctcttccagcacccactcaaccagttcctctgtttctggccgaggaataaacactgggggcaccatccttaggctgagcccctggaagtcccactctccaaggatgtactgcaccggcatcctctgcaatcgacggctactcagctcccggatacactgtagttgctgagaggtcaagggctgggtccaaagtgccggcctcaggctctgaaatgttttggctccaaggacatgagccacgatgtactcactggattcccgggcctcagggatacccctcttctcaaagaccccagtccagtggctgaccagttctatggcactggataacccagccagaggtggttggggttgccatgagctgaaggcccagccccgggtacttcccctcctccctgggccagacaggagggcccacagcattcggccccaaagctccatgtctcagggaaaggttctccagagtgcttccaggttcccaagtctgctttatgatgtcagctgctgaggtgagtgctgagagtggcccctggacccagctgggtggagatggagaggtcacaagctctggtgccccaaaatggctctggtcctcagatatagttggttgccaccctgcctgaaaggctgccccacccacccaccagccggagaagctgccccgaact

SEQ ID NO: 13706 - RNA, 5977 nt, Homo sapiens
  source 1..5977: mol_type = other RNA
gctgggattacaggcatgagccaccatgcccagctgagaagcaaacttctatcttgtacaagcaattgctgtttggggacacagccaacctcatacatatgaactaatgcatgccaagttttaatttccttaactgaaaaggctgatgcaaatgacatattgcacctggtggcaggcagctacatctactgctaaaatgacataagatagaagaagttttctgtagagaacattgtgtgtcacaaacagtgacattttcaaaagtgcttaattcaatatgacttcccagcggcaaagcttgcacctatggttttaggaaaacaacaacaaaaagtttagtctagcttaagatgcaaaatgactgacaaagtccctccccacaagagaactgtaacgagcaatttaaacaaatcaaaaatggtttgttttatttacaatactcaatgcatcttatgagtaacatatttgcattccctaagtcttttggaaagtaattccagtttgtgcagtgagtttacaggaaaatcttaaagatatctagtagacatcttaaacctaaactctaaattttgaaagatatttcacactatattaatagaggactgtttttaattaagaaaaactaaactctgtaaatattgccctccagtatctttaatgcaaatataaaccagattagcctatgaaataagaccactagatttgggtgaattattctgacctcccctccccaataaaatgcatgcataaagtaaacatggtaaattacatcaatcacattttaatacttttttttttggactctctcaactgttgtttgctcaattgtcggtacagataggtaggattccagtctggagaaacccctaaaccactacaccctgcctcagagtagggaagaattttcagtatgtatgtggagacaggctggattagggagccttttgagtggcttctctaggatacctttcttgctaacatgagcaaggttcccctccaggcctgataaagcctgaagaggttagttatttccctactagttctggaagcatcttattcatgccaccataggaggctgtcttcccctgctcctccctgaatcaccacctagattttagtgctttctgagttgatgatggaaaccagttcctgttcaggtgccagaaacttttttttttttgagattgagtctcgctctttcatgctggagtgcagtggtgcgatctcagctcactgcaacctccaccccccgggttcaagcgattctctgcctcaacctcctgagtagctgggattacaggcgcccactaccacacccatctactttttgcaaattttgtagagatggggtttcaccatattggccaggctggtctcaaactcctgacctcaggtgatccacctgcctcagcctcccaaagtgctaggattacaggcgtgagccaccgtgccagaaactgtttttatgtcacataaagatctatgaaacaaggtaaaaggtaattaaaatactttgtgacagagtttgcacctcatgcatgtgaaagagaatgtaattaattttatcatttatatagctgccatcttttttttttttttgagacggagtctccttctgttgcccaggctggagtgcagtggcacgatcttggctttgcaaactccgtctcctgggttcaaatgattctctgccttagcctcctgagtagctgggattacaggagcccaccaccacacccagctaatttttttttttgtatttttagtaaagatggggtttcaccctcttggccaggctggtcttgaactcctgacctcgtgatccacctgcctcggcctcccaaagtgctgggattacagacgtgagccactgcacccggccagctgccatctcttaaaacaaaatccaagtcctagctcttgagccataaagaagaaatagaggtatctctatactggatccacctcaacttagcaacgcatctctgcatctccacaatgccattctcctcaaaacatctgctgtctttaacatctggcataggtggtagaatggggagatactaggctgcagaaataaaatccaacgtttgacaaagccaacagaattttgagataaagaaatggtgaggtagagttgagagagttcaattatattgttgagcacagaccatttggcacattctaaaattagattccctatcaacttctcctttgtggtacctttacaaaatgctgacaccttaggaatcctccaacacctatgtaaagctaacagaataaagtcatttgaagaaattcatccttggctctttagctattatctacccccatattgaagcaaataaaaaacaatgctatccatttgctgaatttatttaaacaagtcaatttagaaataccatagaattaaacaaaacttctgacatgtaaacatactgccatgttcctgaaacagatgttaacacctgataaaagttaataatctcttgttaggaaagctgtccattaataaggccagtcttcagcaaaactaaaaccattttgttcgtttagctttcctagtctgacaacgcaatactgttgaaccacagtcaaatataatgacaacattggatggatagatcagtaccattggttacagctgttaaacaggttcgttcttggcgccacataaaaacaagccaatcacatcgaataaatcatggcttttttttctttatcacaattcactaagtgatgttaattatggtccttgtcaaacacgtttggtaaaggctatttacagtgtacatggctgagcatgcactatttatagttacaaagatacctgccagtttattacaatagaattacacagtgcctgaaaatggtgaaacatctcacacatcatttaaatcaatataatttcaagcaggaaacgttccttatttgaccacaattgcaataattacatgaaaattcttataaaaacatgaatctccttcaagaaattgatgcatattctacgcactacaggttaaggcagtaaaaaaatgtattcctgataactggaggtgttgacaatgtcaattaaagctgtctgactctagtttttcattctccatcatataccaaaagtttgtgaatgatttcatttttaaagtcaacaaagtattagtaactaagaagagttgaagctggaaaaaagtaattgctagggaagggaaaaatgtaaattggattttgcctgaaagttttcaaatcataaacaatagcattatttatgagtctaagccttaaatgtataaaacaaatacatatagttcacttttcttaatttaaaatatactgtactttgaacaattcaagtaatgtaagactatcaaaaataacttcataagccatacacaagtgtcaactgcattttcagtattttaagaactttttaaaaattgtaaactaaaccatgacagtttagttaaacaaatgataaatgactttttatttgcacttgtgatttctttaatacaaattgctaccaacaaatatgtaaagatatggcaggttatgcatttgatcaaagcactttgatttaagcataaaacagattcaaatggtacaagttctgtgcataagatccaaggaattgcttactaatctgtaggcaaccctctttctaatcagaatcctttattcctcggctgcagatgagatagggcacaatctgttgtaaacagggcactgttgttaaaccaggataatattcttaaattaagatcgttcttgttctattaaaaagactttcccaagtgtcttccatcactgagtatattctgctgacctcttaatttcataaattaactttcttttgattccatttttatggtggtgtccgcagttttgttttaaaaattggtttaaatttatataaaactctgtacatgttcacaaattattgcataaacagcataatcttcaagacaagtgtttgcaaacacatgtccaattcaggaaaaaaaatttcacgtttctcgtctggcttttttcttcttttttatttgtttgggagattcccagctagtttcagacttggtctgtgaaggaggcacactattttgcttggtatttgacttggatttatctgtctcttgtagtattggcggcacttgggaagagctcttgtcagaatcactttttgataagattacagatggctcggtagaagtagcaggtggaagagtcttgataggctggctatttttgacgagtacttcggctggatcactagtgcttatggtcttcaaggaaaaagctttttcctgttttggacgggttttagaggtattcactggaaggtcttctctaatctctttttctaattcttctgtgtcctgtgcagtagagttatcttcaccttgcttcttctttttcttttttttctttttggatttcccagttggaagagctccctctcccttttctttatcatcatctgagaccttttgatcatcaggaattggttcctgggactttagaagtgaagctctttcttcgtctacccaattgccccactcttctgctggtgcattccaatcagagttgggatcagcagaagacagaccatcaatgccagaaaatattgaacggtcactccaactccttccccagtcttttccatttgtattagcatctccagtgtcttgactccaggcagatggctcagttttcctctttcctgcagaagcaggtgaaacggagttccacttctcctcacctgcactgatctgtgaggagagttttacagacttttcattccagcctcctccattgacagtgaggttttcattcaatcctgaagaaacctgaagtgtagaatctccttttccagatttaaagttgctaacttgaacatttagatgagaatcacctttattcttcttggaaccaacaggaaatgatgcggttgtaagttgctcggtggtaactgtgatggtattttctatcccagggatagttgaatccaatgaaccagaatcagtcagcaccttatcacgtttacgctgctgtcgtttctctctgtgactaattttagtttcccaggctccttcatcaacttcctttccatcatggcgtgaactgttttgcactgctttagcatctgactttgatttcttcttatttttctttgacttttcatttttcttgtcaatctctggtggctgctttgctgttacactttgaggtgttcgaacagcttcaccctcagccacttcaacagtccgcccatttggtttgggcttctcggacagtttcttccggttcttcttcttctgttcctcgctccggagattcttcagcaaggccaggtcgtcgggggccgcggccggcacggccgccgcctcctcccgcttgcggggcgggctcctccgctttttgcgggcgccggcgcaagccgcggcccagccgtagcccagcagaaacagcagcagcagcccgagcgcgccagtgcccaccaggatcacccagccggggtaccgtttcggctccagccccaggtcgaggcccagctcggtgcgcagaaagcctaggccgaccgagagcatttcccgcagccgggccgagccctcctcggcctgctgggccagctcgtcctgccagctccgtgcagccatcttccctcccgtcagagggactcgcaggatgacgccggggcgcggagacgcagtggaatagtcgagggaagcgaggaagggccgggccgggtaacctcaggccgagcgcatcgcggccgtccctcgcgccggagccggggatcggccgctgccaccgcggggagggcggaggggtctcccaggttccccgctgtcagcctcactccgccgccgccaggagacccgggaggcgggagggagtgtctccagtggcggccgctaagcggcgtctcggcgccagcgccaggccccgctgtcctccctcggcggaacaatggcggctt

SEQ ID NO: 13707 - RNA, 5911 nt, Homo sapiens
  source 1..5911: mol_type = other RNA
gctgggattacaggcatgagccaccatgcccagctgagaagcaaacttctatcttgtacaagcaattgctgtttggggacacagccaacctcatacatatgaactaatgcatgccaagttttaatttccttaactgaaaaggctgatgcaaatgacatattgcacctggtggcaggcagctacatctactgctaaaatgacataagatagaagaagttttctgtagagaacattgtgtgtcacaaacagtgacattttcaaaagtgcttaattcaatatgacttcccagcggcaaagcttgcacctatggttttaggaaaacaacaacaaaaagtttagtctagcttaagatgcaaaatgactgacaaagtccctccccacaagagaactgtaacgagcaatttaaacaaatcaaaaatggtttgttttatttacaatactcaatgcatcttatgagtaacatatttgcattccctaagtcttttggaaagtaattccagtttgtgcagtgagtttacaggaaaatcttaaagatatctagtagacatcttaaacctaaactctaaattttgaaagatatttcacactatattaatagaggactgtttttaattaagaaaaactaaactctgtaaatattgccctccagtatctttaatgcaaatataaaccagattagcctatgaaataagaccactagatttgggtgaattattctgacctcccctccccaataaaatgcatgcataaagtaaacatggtaaattacatcaatcacattttaatacttttttttttggactctctcaactgttgtttgctcaattgtcggtacagataggtaggattccagtctggagaaacccctaaaccactacaccctgcctcagagtagggaagaattttcagtatgtatgtggagacaggctggattagggagccttttgagtggcttctctaggatacctttcttgctaacatgagcaaggttcccctccaggcctgataaagcctgaagaggttagttatttccctactagttctggaagcatcttattcatgccaccataggaggctgtcttcccctgctcctccctgaatcaccacctagattttagtgctttctgagttgatgatggaaaccagttcctgttcaggtgccagaaacttttttttttttgagattgagtctcgctctttcatgctggagtgcagtggtgcgatctcagctcactgcaacctccaccccccgggttcaagcgattctctgcctcaacctcctgagtagctgggattacaggcgcccactaccacacccatctactttttgcaaattttgtagagatggggtttcaccatattggccaggctggtctcaaactcctgacctcaggtgatccacctgcctcagcctcccaaagtgctaggattacaggcgtgagccaccgtgccagaaactgtttttatgtcacataaagatctatgaaacaaggtaaaaggtaattaaaatactttgtgacagagtttgcacctcatgcatgtgaaagagaatgtaattaattttatcatttatatagctgccatcttttttttttttttgagacggagtctccttctgttgcccaggctggagtgcagtggcacgatcttggctttgcaaactccgtctcctgggttcaaatgattctctgccttagcctcctgagtagctgggattacaggagcccaccaccacacccagctaatttttttttttgtatttttagtaaagatggggtttcaccctcttggccaggctggtcttgaactcctgacctcgtgatccacctgcctcggcctcccaaagtgctgggattacagacgtgagccactgcacccggccagctgccatctcttaaaacaaaatccaagtcctagctcttgagccataaagaagaaatagaggtatctctatactggatccacctcaacttagcaacgcatctctgcatctccacaatgccattctcctcaaaacatctgctgtctttaacatctggcataggtggtagaatggggagatactaggctgcagaaataaaatccaacgtttgacaaagccaacagaattttgagataaagaaatggtgaggtagagttgagagagttcaattatattgttgagcacagaccatttggcacattctaaaattagattccctatcaacttctcctttgtggtacctttacaaaatgctgacaccttaggaatcctccaacacctatgtaaagctaacagaataaagtcatttgaagaaattcatccttggctctttagctattatctacccccatattgaagcaaataaaaaacaatgctatccatttgctgaatttatttaaacaagtcaatttagaaataccatagaattaaacaaaacttctgacatgtaaacatactgccatgttcctgaaacagatgttaacacctgataaaagttaataatctcttgttaggaaagctgtccattaataaggccagtcttcagcaaaactaaaaccattttgttcgtttagctttcctagtctgacaacgcaatactgttgaaccacagtcaaatataatgacaacattggatggatagatcagtaccattggttacagctgttaaacaggttcgttcttggcgccacataaaaacaagccaatcacatcgaataaatcatggcttttttttctttatcacaattcactaagtgatgttaattatggtccttgtcaaacacgtttggtaaaggctatttacagtgtacatggctgagcatgcactatttatagttacaaagatacctgccagtttattacaatagaattacacagtgcctgaaaatggtgaaacatctcacacatcatttaaatcaatataatttcaagcaggaaacgttccttatttgaccacaattgcaataattacatgaaaattcttataaaaacatgaatctccttcaagaaattgatgcatattctacgcactacaggttaaggcagtaaaaaaatgtattcctgataactggaggtgttgacaatgtcaattaaagctgtctgactctagtttttcattctccatcatataccaaaagtttgtgaatgatttcatttttaaagtcaacaaagtattagtaactaagaagagttgaagctggaaaaaagtaattgctagggaagggaaaaatgtaaattggattttgcctgaaagttttcaaatcataaacaatagcattatttatgagtctaagccttaaatgtataaaacaaatacatatagttcacttttcttaatttaaaatatactgtactttgaacaattcaagtaatgtaagactatcaaaaataacttcataagccatacacaagtgtcaactgcattttcagtattttaagaactttttaaaaattgtaaactaaaccatgacagtttagttaaacaaatgataaatgactttttatttgcacttgtgatttctttaatacaaattgctaccaacaaatatgtaaagatatggcaggttatgcatttgatcaaagcactttgatttaagcataaaacagattcaaatggtacaagttctgtgcataagatccaaggaattgcttactaatctgtaggcaaccctctttctaatcagaatcctttattcctcggctgcagatgagatagggcacaatctgttgtaaacagggcactgttgttaaaccaggataatattcttaaattaagatcgttcttgttctattaaaaagactttcccaagtgtcttccatcactgagtatattctgctgacctcttaatttcataaattaactttcttttgattccatttttatggtggtgtccgcagttttgttttaaaaattggtttaaatttatataaaactctgtacatgttcacaaattattgcataaacagcataatcttcaagacaagtgtttgcaaacacatgtccaattcaggaaaaaaaatttcacgtttctcgtctggcttttttcttcttttttatttgtttgggagattcccagctagtttcagacttggtctgtgaaggaggcacactattttgcttggtatttgacttggatttatctgtctcttgtagtattggcggcacttgggaagagctcttgtcagaatcactttttgataagattacagatggctcggtagaagtagcaggtggaagagtcttgataggctggctatttttgacgagtacttcggctggatcactagtgcttatggtcttcaaggaaaaagctttttcctgttttggacgggttttagaggtattcactggaaggtcttctctaatctctttttctaattcttctgtgtcctgtgcagtagagttatcttcaccttgcttcttctttttcttttttttctttttggatttcccagttggaagagctccctctcccttttctttatcatcatctgagaccttttgatcatcaggaattggttcctgggactttagaagtgaagctctttcttcgtctacccaattgccccactcttctgctggtgcattccaatcagagttgggatcagcagaagacagaccatcaatgccagaaaatattgaacggtcactccaactccttccccagtcttttccatttgtattagcatctccagtgtcttgactccaggcagatggctcagttttcctctttcctgcagaagcaggtgaaacggagttccacttctcctcacctgcactgatctgtgaggagagttttacagacttttcattccagcctcctccattgacagtgaggttttcattcaatcctgaagaaactttattcttcttggaaccaacaggaaatgatgcggttgtaagttgctcggtggtaactgtgatggtattttctatcccagggatagttgaatccaatgaaccagaatcagtcagcaccttatcacgtttacgctgctgtcgtttctctctgtgactaattttagtttcccaggctccttcatcaacttcctttccatcatggcgtgaactgttttgcactgctttagcatctgactttgatttcttcttatttttctttgacttttcatttttcttgtcaatctctggtggctgctttgctgttacactttgaggtgttcgaacagcttcaccctcagccacttcaacagtccgcccatttggtttgggcttctcggacagtttcttccggttcttcttcttctgttcctcgctccggagattcttcagcaaggccaggtcgtcgggggccgcggccggcacggccgccgcctcctcccgcttgcggggcgggctcctccgctttttgcgggcgccggcgcaagccgcggcccagccgtagcccagcagaaacagcagcagcagcccgagcgcgccagtgcccaccaggatcacccagccggggtaccgtttcggctccagccccaggtcgaggcccagctcggtgcgcagaaagcctaggccgaccgagagcatttcccgcagccgggccgagccctcctcggcctgctgggccagctcgtcctgccagctccgtgcagccatcttccctcccgtcagagggactcgcaggatgacgccggggcgcggagacgcagtggaatagtcgagggaagcgaggaagggccgggccgggtaacctcaggccgagcgcatcgcggccgtccctcgcgccggagccggggatcggccgctgccaccgcggggagggcggaggggtctcccaggttccccgctgtcagcctcactccgccgccgccaggagacccgggaggcgggagggagtgtctccagtggcggccgctaagcggcgtctcggcgccagcgccaggccccgctgtcctccctcggcggaacaatggcggctt

SEQ ID NO: 13708 - RNA, 6076 nt, Homo sapiens
  source 1..6076: mol_type = other RNA
gctgggattacaggcatgagccaccatgcccagctgagaagcaaacttctatcttgtacaagcaattgctgtttggggacacagccaacctcatacatatgaactaatgcatgccaagttttaatttccttaactgaaaaggctgatgcaaatgacatattgcacctggtggcaggcagctacatctactgctaaaatgacataagatagaagaagttttctgtagagaacattgtgtgtcacaaacagtgacattttcaaaagtgcttaattcaatatgacttcccagcggcaaagcttgcacctatggttttaggaaaacaacaacaaaaagtttagtctagcttaagatgcaaaatgactgacaaagtccctccccacaagagaactgtaacgagcaatttaaacaaatcaaaaatggtttgttttatttacaatactcaatgcatcttatgagtaacatatttgcattccctaagtcttttggaaagtaattccagtttgtgcagtgagtttacaggaaaatcttaaagatatctagtagacatcttaaacctaaactctaaattttgaaagatatttcacactatattaatagaggactgtttttaattaagaaaaactaaactctgtaaatattgccctccagtatctttaatgcaaatataaaccagattagcctatgaaataagaccactagatttgggtgaattattctgacctcccctccccaataaaatgcatgcataaagtaaacatggtaaattacatcaatcacattttaatacttttttttttggactctctcaactgttgtttgctcaattgtcggtacagataggtaggattccagtctggagaaacccctaaaccactacaccctgcctcagagtagggaagaattttcagtatgtatgtggagacaggctggattagggagccttttgagtggcttctctaggatacctttcttgctaacatgagcaaggttcccctccaggcctgataaagcctgaagaggttagttatttccctactagttctggaagcatcttattcatgccaccataggaggctgtcttcccctgctcctccctgaatcaccacctagattttagtgctttctgagttgatgatggaaaccagttcctgttcaggtgccagaaacttttttttttttgagattgagtctcgctctttcatgctggagtgcagtggtgcgatctcagctcactgcaacctccaccccccgggttcaagcgattctctgcctcaacctcctgagtagctgggattacaggcgcccactaccacacccatctactttttgcaaattttgtagagatggggtttcaccatattggccaggctggtctcaaactcctgacctcaggtgatccacctgcctcagcctcccaaagtgctaggattacaggcgtgagccaccgtgccagaaactgtttttatgtcacataaagatctatgaaacaaggtaaaaggtaattaaaatactttgtgacagagtttgcacctcatgcatgtgaaagagaatgtaattaattttatcatttatatagctgccatcttttttttttttttgagacggagtctccttctgttgcccaggctggagtgcagtggcacgatcttggctttgcaaactccgtctcctgggttcaaatgattctctgccttagcctcctgagtagctgggattacaggagcccaccaccacacccagctaatttttttttttgtatttttagtaaagatggggtttcaccctcttggccaggctggtcttgaactcctgacctcgtgatccacctgcctcggcctcccaaagtgctgggattacagacgtgagccactgcacccggccagctgccatctcttaaaacaaaatccaagtcctagctcttgagccataaagaagaaatagaggtatctctatactggatccacctcaacttagcaacgcatctctgcatctccacaatgccattctcctcaaaacatctgctgtctttaacatctggcataggtggtagaatggggagatactaggctgcagaaataaaatccaacgtttgacaaagccaacagaattttgagataaagaaatggtgaggtagagttgagagagttcaattatattgttgagcacagaccatttggcacattctaaaattagattccctatcaacttctcctttgtggtacctttacaaaatgctgacaccttaggaatcctccaacacctatgtaaagctaacagaataaagtcatttgaagaaattcatccttggctctttagctattatctacccccatattgaagcaaataaaaaacaatgctatccatttgctgaatttatttaaacaagtcaatttagaaataccatagaattaaacaaaacttctgacatgtaaacatactgccatgttcctgaaacagatgttaacacctgataaaagttaataatctcttgttaggaaagctgtccattaataaggccagtcttcagcaaaactaaaaccattttgttcgtttagctttcctagtctgacaacgcaatactgttgaaccacagtcaaatataatgacaacattggatggatagatcagtaccattggttacagctgttaaacaggttcgttcttggcgccacataaaaacaagccaatcacatcgaataaatcatggcttttttttctttatcacaattcactaagtgatgttaattatggtccttgtcaaacacgtttggtaaaggctatttacagtgtacatggctgagcatgcactatttatagttacaaagatacctgccagtttattacaatagaattacacagtgcctgaaaatggtgaaacatctcacacatcatttaaatcaatataatttcaagcaggaaacgttccttatttgaccacaattgcaataattacatgaaaattcttataaaaacatgaatctccttcaagaaattgatgcatattctacgcactacaggttaaggcagtaaaaaaatgtattcctgataactggaggtgttgacaatgtcaattaaagctgtctgactctagtttttcattctccatcatataccaaaagtttgtgaatgatttcatttttaaagtcaacaaagtattagtaactaagaagagttgaagctggaaaaaagtaattgctagggaagggaaaaatgtaaattggattttgcctgaaagttttcaaatcataaacaatagcattatttatgagtctaagccttaaatgtataaaacaaatacatatagttcacttttcttaatttaaaatatactgtactttgaacaattcaagtaatgtaagactatcaaaaataacttcataagccatacacaagtgtcaactgcattttcagtattttaagaactttttaaaaattgtaaactaaaccatgacagtttagttaaacaaatgataaatgactttttatttgcacttgtgatttctttaatacaaattgctaccaacaaatatgtaaagatatggcaggttatgcatttgatcaaagcactttgatttaagcataaaacagattcaaatggtacaagttctgtgcataagatccaaggaattgcttactaatctgtaggcaaccctctttctaatcagaatcctttattcctcggctgcagatgagatagggcacaatctgttgtaaacagggcactgttgttaaaccaggataatattcttaaattaagatcgttcttgttctattaaaaagactttcccaagtgtcttccatcactgagtatattctgctgacctcttaatttcataaattaactttcttttgattccatttttatggtggtgtccgcagttttgttttaaaaattggtttaaatttatataaaactctgtacatgttcacaaattattgcataaacagcataatcttcaagacaagtgtttgcaaacacatgtccaattcaggaaaaaaaatttcacgtttctcgtctggcttttttcttcttttttatttgtttgggagattcccagctagtttcagacttggtctgtgaaggaggcacactattttgcttggtatttgacttggatttatctgtctcttgtagtattggcggcacttgggaagagctcttgtcagaatcactttttgataagattacagatggctcggtagaagtagcaggtggaagagtcttgataggctggctatttttgacgagtacttcggctggatcactagtgcttatggtcttcaaggaaaaagctttttcctgttttggacgggttttagaggtattcactggaaggtcttctctaatctctttttctaattcttctgtgtcctgtgcagtagagttatcttcaccttgcttcttctttttcttttttttctttttggatttcccagttggaagagctccctctcccttttctttatcatcatctgagaccttttgatcatcaggaattggttcctgggactttagaagtgaagctctttcttcgtctacccaattgccccactcttctgctggtgcattccaatcagagttgggatcagcagaagacagaccatttaacccagaccattcatcatcgatatagggttgattacggctaacatcccactgataatcagaagtggtagactgagaaactggctcagcagtagacccaatgccagaaaatattgaacggtcactccaactccttccccagtcttttccatttgtattagcatctccagtgtcttgactccaggcagatggctcagttttcctctttcctgcagaagcaggtgaaacggagttccacttctcctcacctgcactgatctgtgaggagagttttacagacttttcattccagcctcctccattgacagtgaggttttcattcaatcctgaagaaacctgaagtgtagaatctccttttccagatttaaagttgctaacttgaacatttagatgagaatcacctttattcttcttggaaccaacaggaaatgatgcggttgtaagttgctcggtggtaactgtgatggtattttctatcccagggatagttgaatccaatgaaccagaatcagtcagcaccttatcacgtttacgctgctgtcgtttctctctgtgactaattttagtttcccaggctccttcatcaacttcctttccatcatggcgtgaactgttttgcactgctttagcatctgactttgatttcttcttatttttctttgacttttcatttttcttgtcaatctctggtggctgctttgctgttacactttgaggtgttcgaacagcttcaccctcagccacttcaacagtccgcccatttggtttgggcttctcggacagtttcttccggttcttcttcttctgttcctcgctccggagattcttcagcaaggccaggtcgtcgggggccgcggccggcacggccgccgcctcctcccgcttgcggggcgggctcctccgctttttgcgggcgccggcgcaagccgcggcccagccgtagcccagcagaaacagcagcagcagcccgagcgcgccagtgcccaccaggatcacccagccggggtaccgtttcggctccagccccaggtcgaggcccagctcggtgcgcagaaagcctaggccgaccgagagcatttcccgcagccgggccgagccctcctcggcctgctgggccagctcgtcctgccagctccgtgcagccatcttccctcccgtcagagggactcgcaggatgacgccggggcgcggagacgcagtggaatagtcgagggaagcgaggaagggccgggccgggtaacctcaggccgagcgcatcgcggccgtccctcgcgccggagccggggatcggccgctgccaccgcggggagggcggaggggtctcccaggttccccgctgtcagcctcactccgccgccgccaggagacccgggaggcgggagggagtgtctccagtggcggccgctaagcggcgtctcggcgccagcgccaggccccgctgtcctccctcggcggaacaatggcggctt

SEQ ID NO: 13709 - RNA, 6010 nt, Homo sapiens
  source 1..6010: mol_type = other RNA
gctgggattacaggcatgagccaccatgcccagctgagaagcaaacttctatcttgtacaagcaattgctgtttggggacacagccaacctcatacatatgaactaatgcatgccaagttttaatttccttaactgaaaaggctgatgcaaatgacatattgcacctggtggcaggcagctacatctactgctaaaatgacataagatagaagaagttttctgtagagaacattgtgtgtcacaaacagtgacattttcaaaagtgcttaattcaatatgacttcccagcggcaaagcttgcacctatggttttaggaaaacaacaacaaaaagtttagtctagcttaagatgcaaaatgactgacaaagtccctccccacaagagaactgtaacgagcaatttaaacaaatcaaaaatggtttgttttatttacaatactcaatgcatcttatgagtaacatatttgcattccctaagtcttttggaaagtaattccagtttgtgcagtgagtttacaggaaaatcttaaagatatctagtagacatcttaaacctaaactctaaattttgaaagatatttcacactatattaatagaggactgtttttaattaagaaaaactaaactctgtaaatattgccctccagtatctttaatgcaaatataaaccagattagcctatgaaataagaccactagatttgggtgaattattctgacctcccctccccaataaaatgcatgcataaagtaaacatggtaaattacatcaatcacattttaatacttttttttttggactctctcaactgttgtttgctcaattgtcggtacagataggtaggattccagtctggagaaacccctaaaccactacaccctgcctcagagtagggaagaattttcagtatgtatgtggagacaggctggattagggagccttttgagtggcttctctaggatacctttcttgctaacatgagcaaggttcccctccaggcctgataaagcctgaagaggttagttatttccctactagttctggaagcatcttattcatgccaccataggaggctgtcttcccctgctcctccctgaatcaccacctagattttagtgctttctgagttgatgatggaaaccagttcctgttcaggtgccagaaacttttttttttttgagattgagtctcgctctttcatgctggagtgcagtggtgcgatctcagctcactgcaacctccaccccccgggttcaagcgattctctgcctcaacctcctgagtagctgggattacaggcgcccactaccacacccatctactttttgcaaattttgtagagatggggtttcaccatattggccaggctggtctcaaactcctgacctcaggtgatccacctgcctcagcctcccaaagtgctaggattacaggcgtgagccaccgtgccagaaactgtttttatgtcacataaagatctatgaaacaaggtaaaaggtaattaaaatactttgtgacagagtttgcacctcatgcatgtgaaagagaatgtaattaattttatcatttatatagctgccatcttttttttttttttgagacggagtctccttctgttgcccaggctggagtgcagtggcacgatcttggctttgcaaactccgtctcctgggttcaaatgattctctgccttagcctcctgagtagctgggattacaggagcccaccaccacacccagctaatttttttttttgtatttttagtaaagatggggtttcaccctcttggccaggctggtcttgaactcctgacctcgtgatccacctgcctcggcctcccaaagtgctgggattacagacgtgagccactgcacccggccagctgccatctcttaaaacaaaatccaagtcctagctcttgagccataaagaagaaatagaggtatctctatactggatccacctcaacttagcaacgcatctctgcatctccacaatgccattctcctcaaaacatctgctgtctttaacatctggcataggtggtagaatggggagatactaggctgcagaaataaaatccaacgtttgacaaagccaacagaattttgagataaagaaatggtgaggtagagttgagagagttcaattatattgttgagcacagaccatttggcacattctaaaattagattccctatcaacttctcctttgtggtacctttacaaaatgctgacaccttaggaatcctccaacacctatgtaaagctaacagaataaagtcatttgaagaaattcatccttggctctttagctattatctacccccatattgaagcaaataaaaaacaatgctatccatttgctgaatttatttaaacaagtcaatttagaaataccatagaattaaacaaaacttctgacatgtaaacatactgccatgttcctgaaacagatgttaacacctgataaaagttaataatctcttgttaggaaagctgtccattaataaggccagtcttcagcaaaactaaaaccattttgttcgtttagctttcctagtctgacaacgcaatactgttgaaccacagtcaaatataatgacaacattggatggatagatcagtaccattggttacagctgttaaacaggttcgttcttggcgccacataaaaacaagccaatcacatcgaataaatcatggcttttttttctttatcacaattcactaagtgatgttaattatggtccttgtcaaacacgtttggtaaaggctatttacagtgtacatggctgagcatgcactatttatagttacaaagatacctgccagtttattacaatagaattacacagtgcctgaaaatggtgaaacatctcacacatcatttaaatcaatataatttcaagcaggaaacgttccttatttgaccacaattgcaataattacatgaaaattcttataaaaacatgaatctccttcaagaaattgatgcatattctacgcactacaggttaaggcagtaaaaaaatgtattcctgataactggaggtgttgacaatgtcaattaaagctgtctgactctagtttttcattctccatcatataccaaaagtttgtgaatgatttcatttttaaagtcaacaaagtattagtaactaagaagagttgaagctggaaaaaagtaattgctagggaagggaaaaatgtaaattggattttgcctgaaagttttcaaatcataaacaatagcattatttatgagtctaagccttaaatgtataaaacaaatacatatagttcacttttcttaatttaaaatatactgtactttgaacaattcaagtaatgtaagactatcaaaaataacttcataagccatacacaagtgtcaactgcattttcagtattttaagaactttttaaaaattgtaaactaaaccatgacagtttagttaaacaaatgataaatgactttttatttgcacttgtgatttctttaatacaaattgctaccaacaaatatgtaaagatatggcaggttatgcatttgatcaaagcactttgatttaagcataaaacagattcaaatggtacaagttctgtgcataagatccaaggaattgcttactaatctgtaggcaaccctctttctaatcagaatcctttattcctcggctgcagatgagatagggcacaatctgttgtaaacagggcactgttgttaaaccaggataatattcttaaattaagatcgttcttgttctattaaaaagactttcccaagtgtcttccatcactgagtatattctgctgacctcttaatttcataaattaactttcttttgattccatttttatggtggtgtccgcagttttgttttaaaaattggtttaaatttatataaaactctgtacatgttcacaaattattgcataaacagcataatcttcaagacaagtgtttgcaaacacatgtccaattcaggaaaaaaaatttcacgtttctcgtctggcttttttcttcttttttatttgtttgggagattcccagctagtttcagacttggtctgtgaaggaggcacactattttgcttggtatttgacttggatttatctgtctcttgtagtattggcggcacttgggaagagctcttgtcagaatcactttttgataagattacagatggctcggtagaagtagcaggtggaagagtcttgataggctggctatttttgacgagtacttcggctggatcactagtgcttatggtcttcaaggaaaaagctttttcctgttttggacgggttttagaggtattcactggaaggtcttctctaatctctttttctaattcttctgtgtcctgtgcagtagagttatcttcaccttgcttcttctttttcttttttttctttttggatttcccagttggaagagctccctctcccttttctttatcatcatctgagaccttttgatcatcaggaattggttcctgggactttagaagtgaagctctttcttcgtctacccaattgccccactcttctgctggtgcattccaatcagagttgggatcagcagaagacagaccatttaacccagaccattcatcatcgatatagggttgattacggctaacatcccactgataatcagaagtggtagactgagaaactggctcagcagtagacccaatgccagaaaatattgaacggtcactccaactccttccccagtcttttccatttgtattagcatctccagtgtcttgactccaggcagatggctcagttttcctctttcctgcagaagcaggtgaaacggagttccacttctcctcacctgcactgatctgtgaggagagttttacagacttttcattccagcctcctccattgacagtgaggttttcattcaatcctgaagaaactttattcttcttggaaccaacaggaaatgatgcggttgtaagttgctcggtggtaactgtgatggtattttctatcccagggatagttgaatccaatgaaccagaatcagtcagcaccttatcacgtttacgctgctgtcgtttctctctgtgactaattttagtttcccaggctccttcatcaacttcctttccatcatggcgtgaactgttttgcactgctttagcatctgactttgatttcttcttatttttctttgacttttcatttttcttgtcaatctctggtggctgctttgctgttacactttgaggtgttcgaacagcttcaccctcagccacttcaacagtccgcccatttggtttgggcttctcggacagtttcttccggttcttcttcttctgttcctcgctccggagattcttcagcaaggccaggtcgtcgggggccgcggccggcacggccgccgcctcctcccgcttgcggggcgggctcctccgctttttgcgggcgccggcgcaagccgcggcccagccgtagcccagcagaaacagcagcagcagcccgagcgcgccagtgcccaccaggatcacccagccggggtaccgtttcggctccagccccaggtcgaggcccagctcggtgcgcagaaagcctaggccgaccgagagcatttcccgcagccgggccgagccctcctcggcctgctgggccagctcgtcctgccagctccgtgcagccatcttccctcccgtcagagggactcgcaggatgacgccggggcgcggagacgcagtggaatagtcgagggaagcgaggaagggccgggccgggtaacctcaggccgagcgcatcgcggccgtccctcgcgccggagccggggatcggccgctgccaccgcggggagggcggaggggtctcccaggttccccgctgtcagcctcactccgccgccgccaggagacccgggaggcgggagggagtgtctccagtggcggccgctaagcggcgtctcggcgccagcgccaggccccgctgtcctccctcggcggaacaatggcggctt

SEQ ID NO: 13710 - RNA, 6166 nt, Homo sapiens
  source 1..6166: mol_type = other RNA
gctgggattacaggcatgagccaccatgcccagctgagaagcaaacttctatcttgtacaagcaattgctgtttggggacacagccaacctcatacatatgaactaatgcatgccaagttttaatttccttaactgaaaaggctgatgcaaatgacatattgcacctggtggcaggcagctacatctactgctaaaatgacataagatagaagaagttttctgtagagaacattgtgtgtcacaaacagtgacattttcaaaagtgcttaattcaatatgacttcccagcggcaaagcttgcacctatggttttaggaaaacaacaacaaaaagtttagtctagcttaagatgcaaaatgactgacaaagtccctccccacaagagaactgtaacgagcaatttaaacaaatcaaaaatggtttgttttatttacaatactcaatgcatcttatgagtaacatatttgcattccctaagtcttttggaaagtaattccagtttgtgcagtgagtttacaggaaaatcttaaagatatctagtagacatcttaaacctaaactctaaattttgaaagatatttcacactatattaatagaggactgtttttaattaagaaaaactaaactctgtaaatattgccctccagtatctttaatgcaaatataaaccagattagcctatgaaataagaccactagatttgggtgaattattctgacctcccctccccaataaaatgcatgcataaagtaaacatggtaaattacatcaatcacattttaatacttttttttttggactctctcaactgttgtttgctcaattgtcggtacagataggtaggattccagtctggagaaacccctaaaccactacaccctgcctcagagtagggaagaattttcagtatgtatgtggagacaggctggattagggagccttttgagtggcttctctaggatacctttcttgctaacatgagcaaggttcccctccaggcctgataaagcctgaagaggttagttatttccctactagttctggaagcatcttattcatgccaccataggaggctgtcttcccctgctcctccctgaatcaccacctagattttagtgctttctgagttgatgatggaaaccagttcctgttcaggtgccagaaacttttttttttttgagattgagtctcgctctttcatgctggagtgcagtggtgcgatctcagctcactgcaacctccaccccccgggttcaagcgattctctgcctcaacctcctgagtagctgggattacaggcgcccactaccacacccatctactttttgcaaattttgtagagatggggtttcaccatattggccaggctggtctcaaactcctgacctcaggtgatccacctgcctcagcctcccaaagtgctaggattacaggcgtgagccaccgtgccagaaactgtttttatgtcacataaagatctatgaaacaaggtaaaaggtaattaaaatactttgtgacagagtttgcacctcatgcatgtgaaagagaatgtaattaattttatcatttatatagctgccatcttttttttttttttgagacggagtctccttctgttgcccaggctggagtgcagtggcacgatcttggctttgcaaactccgtctcctgggttcaaatgattctctgccttagcctcctgagtagctgggattacaggagcccaccaccacacccagctaatttttttttttgtatttttagtaaagatggggtttcaccctcttggccaggctggtcttgaactcctgacctcgtgatccacctgcctcggcctcccaaagtgctgggattacagacgtgagccactgcacccggccagctgccatctcttaaaacaaaatccaagtcctagctcttgagccataaagaagaaatagaggtatctctatactggatccacctcaacttagcaacgcatctctgcatctccacaatgccattctcctcaaaacatctgctgtctttaacatctggcataggtggtagaatggggagatactaggctgcagaaataaaatccaacgtttgacaaagccaacagaattttgagataaagaaatggtgaggtagagttgagagagttcaattatattgttgagcacagaccatttggcacattctaaaattagattccctatcaacttctcctttgtggtacctttacaaaatgctgacaccttaggaatcctccaacacctatgtaaagctaacagaataaagtcatttgaagaaattcatccttggctctttagctattatctacccccatattgaagcaaataaaaaacaatgctatccatttgctgaatttatttaaacaagtcaatttagaaataccatagaattaaacaaaacttctgacatgtaaacatactgccatgttcctgaaacagatgttaacacctgataaaagttaataatctcttgttaggaaagctgtccattaataaggccagtcttcagcaaaactaaaaccattttgttcgtttagctttcctagtctgacaacgcaatactgttgaaccacagtcaaatataatgacaacattggatggatagatcagtaccattggttacagctgttaaacaggttcgttcttggcgccacataaaaacaagccaatcacatcgaataaatcatggcttttttttctttatcacaattcactaagtgatgttaattatggtccttgtcaaacacgtttggtaaaggctatttacagtgtacatggctgagcatgcactatttatagttacaaagatacctgccagtttattacaatagaattacacagtgcctgaaaatggtgaaacatctcacacatcatttaaatcaatataatttcaagcaggaaacgttccttatttgaccacaattgcaataattacatgaaaattcttataaaaacatgaatctccttcaagaaattgatgcatattctacgcactacaggttaaggcagtaaaaaaatgtattcctgataactggaggtgttgacaatgtcaattaaagctgtctgactctagtttttcattctccatcatataccaaaagtttgtgaatgatttcatttttaaagtcaacaaagtattagtaactaagaagagttgaagctggaaaaaagtaattgctagggaagggaaaaatgtaaattggattttgcctgaaagttttcaaatcataaacaatagcattatttatgagtctaagccttaaatgtataaaacaaatacatatagttcacttttcttaatttaaaatatactgtactttgaacaattcaagtaatgtaagactatcaaaaataacttcataagccatacacaagtgtcaactgcattttcagtattttaagaactttttaaaaattgtaaactaaaccatgacagtttagttaaacaaatgataaatgactttttatttgcacttgtgatttctttaatacaaattgctaccaacaaatatgtaaagatatggcaggttatgcatttgatcaaagcactttgatttaagcataaaacagattcaaatggtacaagttctgtgcataagatccaaggaattgcttactaatctgtaggcaaccctctttctaatcagaatcctttattcctcggctgcagatgagatagggcacaatctgttgtaaacagggcactgttgttaaaccaggataatattcttaaattaagatcgttcttgttctattaaaaagactttcccaagtgtcttccatcactgagtatattctgctgacctcttaatttcataaattaactttcttttgattccatttttatggtggtgtccgcagttttgttttaaaaattggtttaaatttatataaaactctgtacatgttcacaaattattgcataaacagcataatcttcaagacaagtgtttgcaaacacatgtccaattcaggaaaaaaaatttcacgtttctcgtctggcttttttcttcttttttatttgtttgggagattcccagctagtttcagacttggtctgtgaaggaggcacactattttgcttggtatttgacttggatttatctgtctcttgtagtattggcggcacttgggaagagctcttgtcagaatcactttttgataagattacagatggctcggtagaagtagcaggtggaagagtcttgataggctggctatttttgacgagtacttcggctggatcactagtgcttatggtcttcaaggaaaaagctttttcctgttttggacgggttttagaggtattcactggaaggtcttctctaatctctttttctaattcttctgtgtcctgtgcagtagagttatcttcaccttgcttcttctttttcttttttttctttttggatttcccagttggaagagctccctctcccttttctttatcatcatctgagaccttttgatcatcaggaattggttcctgggactttagaagtgaagctctttcttcgtctacccaattgccccactcttctgctggtgcattccaatcagagttgggatcagcagaagacagaccatttaacccagaccattcatcatcgatatagggttgattacggctaacatcccactgataatcagaagtggtagactgagaaactggctcagcagtagacccagaaacagcagagttaagtgtgagagatgcaaaagaagcagaattctgttcagaggtattcattcccctatccacactagaccaagcagcaatgccagaaaatattgaacggtcactccaactccttccccagtcttttccatttgtattagcatctccagtgtcttgactccaggcagatggctcagttttcctctttcctgcagaagcaggtgaaacggagttccacttctcctcacctgcactgatctgtgaggagagttttacagacttttcattccagcctcctccattgacagtgaggttttcattcaatcctgaagaaacctgaagtgtagaatctccttttccagatttaaagttgctaacttgaacatttagatgagaatcacctttattcttcttggaaccaacaggaaatgatgcggttgtaagttgctcggtggtaactgtgatggtattttctatcccagggatagttgaatccaatgaaccagaatcagtcagcaccttatcacgtttacgctgctgtcgtttctctctgtgactaattttagtttcccaggctccttcatcaacttcctttccatcatggcgtgaactgttttgcactgctttagcatctgactttgatttcttcttatttttctttgacttttcatttttcttgtcaatctctggtggctgctttgctgttacactttgaggtgttcgaacagcttcaccctcagccacttcaacagtccgcccatttggtttgggcttctcggacagtttcttccggttcttcttcttctgttcctcgctccggagattcttcagcaaggccaggtcgtcgggggccgcggccggcacggccgccgcctcctcccgcttgcggggcgggctcctccgctttttgcgggcgccggcgcaagccgcggcccagccgtagcccagcagaaacagcagcagcagcccgagcgcgccagtgcccaccaggatcacccagccggggtaccgtttcggctccagccccaggtcgaggcccagctcggtgcgcagaaagcctaggccgaccgagagcatttcccgcagccgggccgagccctcctcggcctgctgggccagctcgtcctgccagctccgtgcagccatcttccctcccgtcagagggactcgcaggatgacgccggggcgcggagacgcagtggaatagtcgagggaagcgaggaagggccgggccgggtaacctcaggccgagcgcatcgcggccgtccctcgcgccggagccggggatcggccgctgccaccgcggggagggcggaggggtctcccaggttccccgctgtcagcctcactccgccgccgccaggagacccgggaggcgggagggagtgtctccagtggcggccgctaagcggcgtctcggcgccagcgccaggccccgctgtcctccctcggcggaacaatggcggctt

SEQ ID NO: 13711 - RNA, 8211 nt, Homo sapiens
  source 1..8211: mol_type = other RNA
gctgggattacaggcatgagccaccatgcccagcttaagaattcttgatttttggaaccttgattataagctgcctgatgtctggaaccaaaacttctgtaacactctattccacgtgtacttacaaaacactctaaacatttattaaacagtttgatgaaggccaaaataagaggcatatgctattctacaacacggtaacactcttcgtcacttaaaataattaagctttgagaacacaaaataaagctttttaaaaaagccattcagaaataggaagcagtttgggaaatgattgtgctacgccaatcaagaaaatgttgtacctcaaacatctgaaggtagcaatctgtttttttctttccctgcagctacccttattggaaacataagggaatataaagtgaaaacaggcaatgtttgcctgtttttatagcttttagccttaccacttttcagtttggggatggaatgcctttggctcagtagattctactggctttggggagctcagaaaggccataatggggcctacaggaagaggaaaaagagagctgacctcttaagggcaggccttaggtacaagaggctttttttaaaaagtgacaaaacttttgaactaaagatggaaaacgtagtctgacaaagaatatttgtgcaactttacagtgccagtaaaatcatgggaaaagcttggatagccatacgtaggtgtttctgaaacatgtcagattttatatatatatatatatatatatatatatttttttttttttttttttttttttttagagagtcttgctttgttacccaggctggagtgcagtggcacaatctcggatcactgcaaatcctccgcctcctgggttcaagcgattctcctgcctcggtctcccaagtagctgggactacaggcgcctgccatcacacccacctaatttatgtttttgctagagatggggtttcaccatgttccatgttagccaggctggtctccaactcctgacttcagattatctgcccgccttggcctcccaaagtgctgggattacaggcgtgagcctccatacccggcccatgtcagatatatttaaaactaagaaagcttgggaaaatctctgccaatgatctccatatcagttaaccccgttccatagagtcagaaaggcagagggtcttagtgcagatgcctgcataaagataaaacgttgcatgttcttggaaaatatggctagaccacccttcccataccatctagctgcagtataaattaacatacccatgtggaaaagtggtatgaatcaagaactacaaaagtgttcatatacccttgactagaaattccacctccagtattttatcctaagaaaataatttatacacaaagacattcattgtggcattatgagatataatctaaactgttcaaaataagtaaaggttatatgaaacatggcacatccataacaatggagtaccataaaattaataatagttgacacagttttaatgacatggaataatgcctgtaggttgcggggaaaaaccccaagatataaattacactgagaatgatgaaactaagtaaaaatatgcagaagtagcaaagacaatggcaaggaagatgcaaaaatatcaagtgattttttctggtgacagaatcataggcaattaattgttatacttttctgtattgtctaaattttccacaataagcatgtactactgacataaacagaaaaaacaaacattattcaaccaggcaagcattaaagaatggacattgggtacagctttatttatttcttttaggaattgcaggttcctaacaaagtaggggtgaggggggtgttacaaaccagtcactaggcaggaacattagactccaaaagcagagaaatgcttaattttcttctacctgtttcaccacattcatgtagaactgtagtaaaaaagatggtgaatcaggctgaatcaatctaaataacaacttaaggctcccaaatcacatgaacctaggaccactaaatccaatgtcagacgtgtttaaatggtgcactgctctacatttttctattatgcaaagagctagaaaataatggtagtgtcattatgacattccatgaaaatgaagaaaatctttcaggaaaaattaagaaaataaaaatgtttactaaagaaagaatggtccggctaagtgcttttttttttttttttttttttaaaccaactgaaggccagagaaatgaaaggcatacccgtgaattaaattaatgctttaaaaaaaattgactttacttaaaatacaaacaaacgtcaactaatgaatactttattggcagaaaaaaaagacaacttggctggaaatgctgagtgtcttggactggtctgaaggaagaacatctgaaaggtctgaatgtcaaagtcagaacagtctctggtcaatcctactttgcttaaaatccaacattttacctttcttcaaattcctcaagactaaggaaaacttggttttataccaagaattatgaatcaacctacacttgctatcccttacatcacattttcattctagcttttctgaaacacattaccagataaatgccatataacctaaattcacctcaatgctttcattttgcctttacaattaccttaggacagatgccaagtttttataacttcaggccagaaaatcctcaagtggctcacctaattgtcagaaagtgagtgagtgacaacagacctcaggcacgaaactattttcagcaccaattacactgtggggggttaccagaacaagaaaaggccttcatagttctaagtgaagaaagataaaaacattttattttggccaggcgcggtggctcacgcctgtaaatcccagcactttgggaggccaaggcaggcggatcacctgaggtcgggagttcgagaccagcctgaccaaaatggagaaaccccgtatctactaaaaatacaaaattagctgggcgtggtgatacatgcctgtaatcccagctactcgggaggctgaggcaggagaatcgcttgaaccctgtaggtggaggttgcggtgagccaagatcgcaccattgcactccatcccgggcaacaagagcaagactcagcctcaaaaaaaaaaaaaaaaaaattgattttaggaggctgacaattacagttcatttcctaagatattccagacaatcactggttggctgacagaatctaggtgacagctaagatcacccctctgaaactcccttatatttggttaagcagaaatctgggctagcaaaataaactactagaaagtcagggtctggataagaaacagtgaccacattaaaggctgacggattaataatcatgatgttgccataaggccaaagtcataaagtactaatgctcaagacagataaacaacgtaagccccaatttcaagatgataaacttcaaagtgtattttttaaaatgcaagttgcctgtatgaaataaattaaaaatttatatgtaatttcagtgtaaaacaccaaaaccgaacattaaaactgttcacagaaaatagaaaaaaaaacaaaaaaacaaatcacaattataaaagcacagagatatcagttataagaaccaagtaaataaactaatttctattaatattttcatttactttataaaactttgttgattaaattgggggagtctctgacaatctaaagggtaacaaaataacaaatatacatcatttctttataagtcataccacacaaaccaagttaagttttttctatctgattacagagtcaataaatattgcatctgtatttagagcagcaacataaaactttattagaaagaaatactatatctggaccaaaaaactgcaacatggtttggaaatctaatgactaagaaggtaaaactggcaactatgtgcaactactgctcgtagatttgggtttgtttcccccccaacatctttaaaataagcagcccccacaaagggataatccattgaataaggagacaatgtagccaaagaagggatttgtggaaaaccatatgaatttaaatcaacataaaaagaacacacaaaggccatggaaacttgagaaggtgaaagaaaaaaaaaaaaaaccccaagcaaggacaagtcagctccttggagctgcaccaactcttaagtaggatgtccctattctaacggaaattgatgagtccacacctgggcacttcagtttgagaaatcaattggttggactggccattaaaaaaaggactttgtttttaaggtagataaagcttagagagagaaagctaaacagaaaagtaccaaatccttgtgaactcaaaaatgatttaggaagtcaaatgaagcaaactaaaaaactggatgaaaatgtttctctaagagtaaaacccagttttctctgtgatttaaaatcaaacaaacacactatagaagagaaattttcaaagtgcacccaataaaacctcagaggttccctggagtgtttggggtagcatggattgagacaggaagtgggttcaggcccatctcccccaacccttcttcactttaattcaaacatttctaattctcttttgtcgtttgtagtttcaggtaagatatcattttaaaaaaatgaaaaaaaaaaaaaatctaatgctgtccctttccctaagtttgaaaatcactgctgagactgaaattacattggtgagaaatatgatcatcataaatctaaaacacattttctatgtagtgctaccaaaatacaaagtttcatcaaatatttcactactattctgtaaaataaatgagaaaattaagttgttgggaagaaattaaattttgttattaccacctcccaaaatctgctcttctgctggctccaagatatcaatatttgatagtgtgaacaaatttctaacaaacattccagtcacaccgtaccccaaagacatttcattcaatggctgcatagtttcttttttgagaaggcaagcctcaaatttatagaaaactctagaatgaaaaatgtacaattactaaaaacataataacacactttatgtcagggcagaatctgcatagtgcttttaaacataatcaccaatgaagagtagccaaatcccagaacttcacacagcactcattagcaaacaacgtcaaagtgtaaatgataagcaggaaaaaaaccaagtaacacgaatgccatttttctttgatgcaatcacgaagaaaagtggaaatgcaggacgaaaagtggaatccaagctttggccacgtactgaaacttcattacttcaatgaaacagagcaaatctccatggaaaggactcattcagcaaacattaagttctttccatatattttttttccttcacgtaaggttaaacagaagttgctgtcattctagaatcagtgattacaattttttttttaattagaaaaaaggttacttgaatatttacataattttattgctctttattttaacaaaaacttttttcactgatttgtagactccatccattaacgtatgaaagtgaaatccatctctcaggaagatacagttatggttgaatgtatctgatgctgagagtacagcataattaagaaaaatccttgcatgtcatttggttcttgttgcagtcttctgtgttcacccctcagaaagcaaaagaatccatctgactttcaataaataccaaattattaaaaaaaaaaaaaaaagaacgtttccacagactagagatccaagaaaaagcagttctgatgaatgattcccagaatcaagtgagtcctcctttagtccaatgagatgatgtcaggaatgttacttccactgctggttatgacccctgtctcactcctgctgctggatgaactaacatgagtactgctttcatgggagctggtggtggtgacagacgtactgcttgctgttaagggtgaggtgagactatccaaaaacataggaggacagtactgctggggatcaactggaataagggaaagaaaatccaaacctgacaatatggcactagcaataataaggcagtcatatttttccttgaaataagctgttttccactccataaatacaaattatttgttttattttgtattcactgttgcacagtatcagaagatgttccaagcttcagttcattattaatatcatttcttctttgttctcctggcaaatctgatgacatgcttgatattggcgtatggtggaatggtactgagtagtctgttaatgaaggcggaatagcagcaggatcaaccgaagtcacactgggcacccttacagaagatggctgatacatgagaacccctttggttgggctgctttgtgtttctgacataaagatgcatttccttttggcaggagggtcttcctcttcgtcagaagagctttctattgtaagatcaataacatctactttcttcttgcttgcctcactggctacagtcactgaacaaggcttactgaggacgcttgaactttctatttttgtacacggttggctggatactttcatagcttctttcttcggtctcattggacaccaagaaccatcttcttggaatttgatctcatctacatcagaacagtcattgagaatttccataaaaagcccatctaatattagactttcataggcagcttttttgtcacacacaggacaaatccaggtgggctttttctcattcatttgtagatagagggcagcatcaaaacactgcagatgtgtacaagtcactgcacggcatgggattgtcagcctcatttttcctaaagggcacatcaaggatacccgaaggctagttgtagcaatttcactatcaggatctgcagtaagtttttctttaattagtgctctggaatgatcagggtttctaatacctttcatttttaatctctgtaataacatggctgatgtaagctgccgtacaagatatacagacatagagtaattcttcccaatttctgatgcccaagaaatggaaatttggtttggcacagctgaagataacctaactaaagatgtaatattcaaggggcgtccagggcgcttctgttcaatcccatttttaggcggtggtgcatagccaggcaaaggaaatagcttcccatttacttttatacatagactatttggatagttatcttcttgagggcaacttgtctctgccaggcaaagtctcaactgaacttggactgtataatctctcctaccacctggcaaaaaatccctggatatgcatatctctctaacttgttgaggtgtcaaagcaaaaataaaaaacttctcttgaaatcgctgaatactgctttgaactaaactcgtgggcttgatgagaacatcaaggacatcataaaagggcagattttttaactgcacatcaggatggacaggaggaattgggggagatggctgctgcatctcaaatgtgggcttagtatcttgaagcagcacagaaccaacaggagaggatggtgagtgaggtgtaactgaagtggaaggcaacgagtggattccagccacggccaagtcaggttctacaggtgatgagccaccatccaaactgaaaaccgatgatttgattgtggataaatcagaaagtccttcaagagttcgtggatatcggcgtctatacaattctcggattttaatctgaaccgcagggctgcagccgctcttcaataaatgcagcgccctcatcaggaggtcatgcttgcgtccacttttattccgtccagcaaagcctagtaatacttgtagttcagaaaccctaaaactagaaaccatattcagaatggctaaaatgaaaaacactgataacaccaaatgctggcgaggatgctgagaaactggatcactccatacattgctggtagggatgtaaaatggtacagccacttgtgaaactttgaaagcattccctttaaaatcaggaacaagatcaggatgcccccatcacagcttctattcaacattgtactggagatccctcaactcttcgaaatccgccattttataccacccgcgggcgccgccgccgctgccgccgcacccactcccgctgccgccaacgacgctgccgccaccacggccgccgccgcctccagcaccatcctgcactgggcgccgcttaagacgccgcggccgccgccgctacagccgggcccgtcacgt

SEQ ID NO: 13712 - RNA, 7758 nt, Homo sapiens
  source 1..7758: mol_type = other RNA
gctgggattacaggcatgagccaccatgcccagcttaagaattcttgatttttggaaccttgattataagctgcctgatgtctggaaccaaaacttctgtaacactctattccacgtgtacttacaaaacactctaaacatttattaaacagtttgatgaaggccaaaataagaggcatatgctattctacaacacggtaacactcttcgtcacttaaaataattaagctttgagaacacaaaataaagctttttaaaaaagccattcagaaataggaagcagtttgggaaatgattgtgctacgccaatcaagaaaatgttgtacctcaaacatctgaaggtagcaatctgtttttttctttccctgcagctacccttattggaaacataagggaatataaagtgaaaacaggcaatgtttgcctgtttttatagcttttagccttaccacttttcagtttggggatggaatgcctttggctcagtagattctactggctttggggagctcagaaaggccataatggggcctacaggaagaggaaaaagagagctgacctcttaagggcaggccttaggtacaagaggctttttttaaaaagtgacaaaacttttgaactaaagatggaaaacgtagtctgacaaagaatatttgtgcaactttacagtgccagtaaaatcatgggaaaagcttggatagccatacgtaggtgtttctgaaacatgtcagattttatatatatatatatatatatatatatatttttttttttttttttttttttttttagagagtcttgctttgttacccaggctggagtgcagtggcacaatctcggatcactgcaaatcctccgcctcctgggttcaagcgattctcctgcctcggtctcccaagtagctgggactacaggcgcctgccatcacacccacctaatttatgtttttgctagagatggggtttcaccatgttccatgttagccaggctggtctccaactcctgacttcagattatctgcccgccttggcctcccaaagtgctgggattacaggcgtgagcctccatacccggcccatgtcagatatatttaaaactaagaaagcttgggaaaatctctgccaatgatctccatatcagttaaccccgttccatagagtcagaaaggcagagggtcttagtgcagatgcctgcataaagataaaacgttgcatgttcttggaaaatatggctagaccacccttcccataccatctagctgcagtataaattaacatacccatgtggaaaagtggtatgaatcaagaactacaaaagtgttcatatacccttgactagaaattccacctccagtattttatcctaagaaaataatttatacacaaagacattcattgtggcattatgagatataatctaaactgttcaaaataagtaaaggttatatgaaacatggcacatccataacaatggagtaccataaaattaataatagttgacacagttttaatgacatggaataatgcctgtaggttgcggggaaaaaccccaagatataaattacactgagaatgatgaaactaagtaaaaatatgcagaagtagcaaagacaatggcaaggaagatgcaaaaatatcaagtgattttttctggtgacagaatcataggcaattaattgttatacttttctgtattgtctaaattttccacaataagcatgtactactgacataaacagaaaaaacaaacattattcaaccaggcaagcattaaagaatggacattgggtacagctttatttatttcttttaggaattgcaggttcctaacaaagtaggggtgaggggggtgttacaaaccagtcactaggcaggaacattagactccaaaagcagagaaatgcttaattttcttctacctgtttcaccacattcatgtagaactgtagtaaaaaagatggtgaatcaggctgaatcaatctaaataacaacttaaggctcccaaatcacatgaacctaggaccactaaatccaatgtcagacgtgtttaaatggtgcactgctctacatttttctattatgcaaagagctagaaaataatggtagtgtcattatgacattccatgaaaatgaagaaaatctttcaggaaaaattaagaaaataaaaatgtttactaaagaaagaatggtccggctaagtgcttttttttttttttttttttttaaaccaactgaaggccagagaaatgaaaggcatacccgtgaattaaattaatgctttaaaaaaaattgactttacttaaaatacaaacaaacgtcaactaatgaatactttattggcagaaaaaaaagacaacttggctggaaatgctgagtgtcttggactggtctgaaggaagaacatctgaaaggtctgaatgtcaaagtcagaacagtctctggtcaatcctactttgcttaaaatccaacattttacctttcttcaaattcctcaagactaaggaaaacttggttttataccaagaattatgaatcaacctacacttgctatcccttacatcacattttcattctagcttttctgaaacacattaccagataaatgccatataacctaaattcacctcaatgctttcattttgcctttacaattaccttaggacagatgccaagtttttataacttcaggccagaaaatcctcaagtggctcacctaattgtcagaaagtgagtgagtgacaacagacctcaggcacgaaactattttcagcaccaattacactgtggggggttaccagaacaagaaaaggccttcatagttctaagtgaagaaagataaaaacattttattttggccaggcgcggtggctcacgcctgtaaatcccagcactttgggaggccaaggcaggcggatcacctgaggtcgggagttcgagaccagcctgaccaaaatggagaaaccccgtatctactaaaaatacaaaattagctgggcgtggtgatacatgcctgtaatcccagctactcgggaggctgaggcaggagaatcgcttgaaccctgtaggtggaggttgcggtgagccaagatcgcaccattgcactccatcccgggcaacaagagcaagactcagcctcaaaaaaaaaaaaaaaaaaattgattttaggaggctgacaattacagttcatttcctaagatattccagacaatcactggttggctgacagaatctaggtgacagctaagatcacccctctgaaactcccttatatttggttaagcagaaatctgggctagcaaaataaactactagaaagtcagggtctggataagaaacagtgaccacattaaaggctgacggattaataatcatgatgttgccataaggccaaagtcataaagtactaatgctcaagacagataaacaacgtaagccccaatttcaagatgataaacttcaaagtgtattttttaaaatgcaagttgcctgtatgaaataaattaaaaatttatatgtaatttcagtgtaaaacaccaaaaccgaacattaaaactgttcacagaaaatagaaaaaaaaacaaaaaaacaaatcacaattataaaagcacagagatatcagttataagaaccaagtaaataaactaatttctattaatattttcatttactttataaaactttgttgattaaattgggggagtctctgacaatctaaagggtaacaaaataacaaatatacatcatttctttataagtcataccacacaaaccaagttaagttttttctatctgattacagagtcaataaatattgcatctgtatttagagcagcaacataaaactttattagaaagaaatactatatctggaccaaaaaactgcaacatggtttggaaatctaatgactaagaaggtaaaactggcaactatgtgcaactactgctcgtagatttgggtttgtttcccccccaacatctttaaaataagcagcccccacaaagggataatccattgaataaggagacaatgtagccaaagaagggatttgtggaaaaccatatgaatttaaatcaacataaaaagaacacacaaaggccatggaaacttgagaaggtgaaagaaaaaaaaaaaaaaccccaagcaaggacaagtcagctccttggagctgcaccaactcttaagtaggatgtccctattctaacggaaattgatgagtccacacctgggcacttcagtttgagaaatcaattggttggactggccattaaaaaaaggactttgtttttaaggtagataaagcttagagagagaaagctaaacagaaaagtaccaaatccttgtgaactcaaaaatgatttaggaagtcaaatgaagcaaactaaaaaactggatgaaaatgtttctctaagagtaaaacccagttttctctgtgatttaaaatcaaacaaacacactatagaagagaaattttcaaagtgcacccaataaaacctcagaggttccctggagtgtttggggtagcatggattgagacaggaagtgggttcaggcccatctcccccaacccttcttcactttaattcaaacatttctaattctcttttgtcgtttgtagtttcaggtaagatatcattttaaaaaaatgaaaaaaaaaaaaaatctaatgctgtccctttccctaagtttgaaaatcactgctgagactgaaattacattggtgagaaatatgatcatcataaatctaaaacacattttctatgtagtgctaccaaaatacaaagtttcatcaaatatttcactactattctgtaaaataaatgagaaaattaagttgttgggaagaaattaaattttgttattaccacctcccaaaatctgctcttctgctggctccaagatatcaatatttgatagtgtgaacaaatttctaacaaacattccagtcacaccgtaccccaaagacatttcattcaatggctgcatagtttcttttttgagaaggcaagcctcaaatttatagaaaactctagaatgaaaaatgtacaattactaaaaacataataacacactttatgtcagggcagaatctgcatagtgcttttaaacataatcaccaatgaagagtagccaaatcccagaacttcacacagcactcattagcaaacaacgtcaaagtgtaaatgataagcaggaaaaaaaccaagtaacacgaatgccatttttctttgatgcaatcacgaagaaaagtggaaatgcaggacgaaaagtggaatccaagctttggccacgtactgaaacttcattacttcaatgaaacagagcaaatctccatggaaaggactcattcagcaaacattaagttctttccatatattttttttccttcacgtaaggttaaacagaagttgctgtcattctagaatcagtgattacaattttttttttaattagaaaaaaggttacttgaatatttacataattttattgctctttattttaacaaaaacttttttcactgatttgtagactccatccattaacgtatgaaagtgaaatccatctctcaggaagatacagttatggttgaatgtatctgatgctgagagtacagcataattaagaaaaatccttgcatgtcatttggttcttgttgcagtcttctgtgttcacccctcagaaagcaaaagaatccatctgactttcaataaataccaaattattaaaaaaaaaaaaaaaagaacgtttccacagactagagatccaagaaaaagcagttctgatgaatgattcccagaatcaagtgagtcctcctttagtccaatgagatgatgtcaggaatgttacttccactgctggttatgacccctgtctcactcctgctgctggatgaactaacatgagtactgctttcatgggagctggtggtggtgacagacgtactgcttgctgttaagggtgaggtgagactatccaaaaacataggaggacagtactgctggggatcaactggaataagggaaagaaaatccaaacctggcaaatctgatgacatgcttgatattggcgtatggtggaatggtactgagtagtctgttaatgaaggcggaatagcagcaggatcaaccgaagtcacactgggcacccttacagaagatggctgatacatgagaacccctttggttgggctgctttgtgtttctgacataaagatgcatttccttttggcaggagggtcttcctcttcgtcagaagagctttctattgtaagatcaataacatctactttcttcttgcttgcctcactggctacagtcactgaacaaggcttactgaggacgcttgaactttctatttttgtacacggttggctggatactttcatagcttctttcttcggtctcattggacaccaagaaccatcttcttggaatttgatctcatctacatcagaacagtcattgagaatttccataaaaagcccatctaatattagactttcataggcagcttttttgtcacacacaggacaaatccaggtgggctttttctcattcatttgtagatagagggcagcatcaaaacactgcagatgtgtacaagtcactgcacggcatgggattgtcagcctcatttttcctaaagggcacatcaaggatacccgaaggctagttgtagcaatttcactatcaggatctgcagtaagtttttctttaattagtgctctggaatgatcagggtttctaatacctttcatttttaatctctgtaataacatggctgatgtaagctgccgtacaagatatacagacatagagtaattcttcccaatttctgatgcccaagaaatggaaatttggtttggcacagctgaagataacctaactaaagatgtaatattcaaggggcgtccagggcgcttctgttcaatcccatttttaggcggtggtgcatagccaggcaaaggaaatagcttcccatttacttttatacatagactatttggatagttatcttcttgagggcaacttgtctctgccaggcaaagtctcaactgaacttggactgtataatctctcctaccacctggcaaaaaatccctaaactcgtgggcttgatgagaacatcaaggacatcataaaagggcagattttttaactgcacatcaggatggacaggaggaattgggggagatggctgctgcatctcaaatgtgggcttagtatcttgaagcagcacagaaccaacaggagaggatggtgagtgaggtgtaactgaagtggaaggcaacgagtggattccagccacggccaagtcaggttctacaggtgatgagccaccatccaaactgaaaaccgatgatttgattgtggataaatcagaaagtccttcaagagttcgtggatatcggcgtctatacaattctcggattttaatctgaaccgcagggctgcagccgctcttcaataaatgcagcgccctcatcaggaggtcatgcttgcgtccacttttattccgtccagcaaagcctagtaatacttgtagttcagaaaccctaaaactagaaaccatattcctcaactcttcgaaatccgccattttataccacccgcgggcgccgccgccgctgccgccgcacccactcccgctgccgccaacgacgctgccgccaccacggccgccgccgcctccagcaccatcctgcactgggcgccgcttaagacgccgcggccgccgccgctacagccgggcccgtcacgt

SEQ ID NO: 13713 - RNA, 7952 nt, Homo sapiens
  source 1..7952: mol_type = other RNA
gctgggattacaggcatgagccaccatgcccagcttaagaattcttgatttttggaaccttgattataagctgcctgatgtctggaaccaaaacttctgtaacactctattccacgtgtacttacaaaacactctaaacatttattaaacagtttgatgaaggccaaaataagaggcatatgctattctacaacacggtaacactcttcgtcacttaaaataattaagctttgagaacacaaaataaagctttttaaaaaagccattcagaaataggaagcagtttgggaaatgattgtgctacgccaatcaagaaaatgttgtacctcaaacatctgaaggtagcaatctgtttttttctttccctgcagctacccttattggaaacataagggaatataaagtgaaaacaggcaatgtttgcctgtttttatagcttttagccttaccacttttcagtttggggatggaatgcctttggctcagtagattctactggctttggggagctcagaaaggccataatggggcctacaggaagaggaaaaagagagctgacctcttaagggcaggccttaggtacaagaggctttttttaaaaagtgacaaaacttttgaactaaagatggaaaacgtagtctgacaaagaatatttgtgcaactttacagtgccagtaaaatcatgggaaaagcttggatagccatacgtaggtgtttctgaaacatgtcagattttatatatatatatatatatatatatatatttttttttttttttttttttttttttagagagtcttgctttgttacccaggctggagtgcagtggcacaatctcggatcactgcaaatcctccgcctcctgggttcaagcgattctcctgcctcggtctcccaagtagctgggactacaggcgcctgccatcacacccacctaatttatgtttttgctagagatggggtttcaccatgttccatgttagccaggctggtctccaactcctgacttcagattatctgcccgccttggcctcccaaagtgctgggattacaggcgtgagcctccatacccggcccatgtcagatatatttaaaactaagaaagcttgggaaaatctctgccaatgatctccatatcagttaaccccgttccatagagtcagaaaggcagagggtcttagtgcagatgcctgcataaagataaaacgttgcatgttcttggaaaatatggctagaccacccttcccataccatctagctgcagtataaattaacatacccatgtggaaaagtggtatgaatcaagaactacaaaagtgttcatatacccttgactagaaattccacctccagtattttatcctaagaaaataatttatacacaaagacattcattgtggcattatgagatataatctaaactgttcaaaataagtaaaggttatatgaaacatggcacatccataacaatggagtaccataaaattaataatagttgacacagttttaatgacatggaataatgcctgtaggttgcggggaaaaaccccaagatataaattacactgagaatgatgaaactaagtaaaaatatgcagaagtagcaaagacaatggcaaggaagatgcaaaaatatcaagtgattttttctggtgacagaatcataggcaattaattgttatacttttctgtattgtctaaattttccacaataagcatgtactactgacataaacagaaaaaacaaacattattcaaccaggcaagcattaaagaatggacattgggtacagctttatttatttcttttaggaattgcaggttcctaacaaagtaggggtgaggggggtgttacaaaccagtcactaggcaggaacattagactccaaaagcagagaaatgcttaattttcttctacctgtttcaccacattcatgtagaactgtagtaaaaaagatggtgaatcaggctgaatcaatctaaataacaacttaaggctcccaaatcacatgaacctaggaccactaaatccaatgtcagacgtgtttaaatggtgcactgctctacatttttctattatgcaaagagctagaaaataatggtagtgtcattatgacattccatgaaaatgaagaaaatctttcaggaaaaattaagaaaataaaaatgtttactaaagaaagaatggtccggctaagtgcttttttttttttttttttttttaaaccaactgaaggccagagaaatgaaaggcatacccgtgaattaaattaatgctttaaaaaaaattgactttacttaaaatacaaacaaacgtcaactaatgaatactttattggcagaaaaaaaagacaacttggctggaaatgctgagtgtcttggactggtctgaaggaagaacatctgaaaggtctgaatgtcaaagtcagaacagtctctggtcaatcctactttgcttaaaatccaacattttacctttcttcaaattcctcaagactaaggaaaacttggttttataccaagaattatgaatcaacctacacttgctatcccttacatcacattttcattctagcttttctgaaacacattaccagataaatgccatataacctaaattcacctcaatgctttcattttgcctttacaattaccttaggacagatgccaagtttttataacttcaggccagaaaatcctcaagtggctcacctaattgtcagaaagtgagtgagtgacaacagacctcaggcacgaaactattttcagcaccaattacactgtggggggttaccagaacaagaaaaggccttcatagttctaagtgaagaaagataaaaacattttattttggccaggcgcggtggctcacgcctgtaaatcccagcactttgggaggccaaggcaggcggatcacctgaggtcgggagttcgagaccagcctgaccaaaatggagaaaccccgtatctactaaaaatacaaaattagctgggcgtggtgatacatgcctgtaatcccagctactcgggaggctgaggcaggagaatcgcttgaaccctgtaggtggaggttgcggtgagccaagatcgcaccattgcactccatcccgggcaacaagagcaagactcagcctcaaaaaaaaaaaaaaaaaaattgattttaggaggctgacaattacagttcatttcctaagatattccagacaatcactggttggctgacagaatctaggtgacagctaagatcacccctctgaaactcccttatatttggttaagcagaaatctgggctagcaaaataaactactagaaagtcagggtctggataagaaacagtgaccacattaaaggctgacggattaataatcatgatgttgccataaggccaaagtcataaagtactaatgctcaagacagataaacaacgtaagccccaatttcaagatgataaacttcaaagtgtattttttaaaatgcaagttgcctgtatgaaataaattaaaaatttatatgtaatttcagtgtaaaacaccaaaaccgaacattaaaactgttcacagaaaatagaaaaaaaaacaaaaaaacaaatcacaattataaaagcacagagatatcagttataagaaccaagtaaataaactaatttctattaatattttcatttactttataaaactttgttgattaaattgggggagtctctgacaatctaaagggtaacaaaataacaaatatacatcatttctttataagtcataccacacaaaccaagttaagttttttctatctgattacagagtcaataaatattgcatctgtatttagagcagcaacataaaactttattagaaagaaatactatatctggaccaaaaaactgcaacatggtttggaaatctaatgactaagaaggtaaaactggcaactatgtgcaactactgctcgtagatttgggtttgtttcccccccaacatctttaaaataagcagcccccacaaagggataatccattgaataaggagacaatgtagccaaagaagggatttgtggaaaaccatatgaatttaaatcaacataaaaagaacacacaaaggccatggaaacttgagaaggtgaaagaaaaaaaaaaaaaaccccaagcaaggacaagtcagctccttggagctgcaccaactcttaagtaggatgtccctattctaacggaaattgatgagtccacacctgggcacttcagtttgagaaatcaattggttggactggccattaaaaaaaggactttgtttttaaggtagataaagcttagagagagaaagctaaacagaaaagtaccaaatccttgtgaactcaaaaatgatttaggaagtcaaatgaagcaaactaaaaaactggatgaaaatgtttctctaagagtaaaacccagttttctctgtgatttaaaatcaaacaaacacactatagaagagaaattttcaaagtgcacccaataaaacctcagaggttccctggagtgtttggggtagcatggattgagacaggaagtgggttcaggcccatctcccccaacccttcttcactttaattcaaacatttctaattctcttttgtcgtttgtagtttcaggtaagatatcattttaaaaaaatgaaaaaaaaaaaaaatctaatgctgtccctttccctaagtttgaaaatcactgctgagactgaaattacattggtgagaaatatgatcatcataaatctaaaacacattttctatgtagtgctaccaaaatacaaagtttcatcaaatatttcactactattctgtaaaataaatgagaaaattaagttgttgggaagaaattaaattttgttattaccacctcccaaaatctgctcttctgctggctccaagatatcaatatttgatagtgtgaacaaatttctaacaaacattccagtcacaccgtaccccaaagacatttcattcaatggctgcatagtttcttttttgagaaggcaagcctcaaatttatagaaaactctagaatgaaaaatgtacaattactaaaaacataataacacactttatgtcagggcagaatctgcatagtgcttttaaacataatcaccaatgaagagtagccaaatcccagaacttcacacagcactcattagcaaacaacgtcaaagtgtaaatgataagcaggaaaaaaaccaagtaacacgaatgccatttttctttgatgcaatcacgaagaaaagtggaaatgcaggacgaaaagtggaatccaagctttggccacgtactgaaacttcattacttcaatgaaacagagcaaatctccatggaaaggactcattcagcaaacattaagttctttccatatattttttttccttcacgtaaggttaaacagaagttgctgtcattctagaatcagtgattacaattttttttttaattagaaaaaaggttacttgaatatttacataattttattgctctttattttaacaaaaacttttttcactgatttgtagactccatccattaacgtatgaaagtgaaatccatctctcaggaagatacagttatggttgaatgtatctgatgctgagagtacagcataattaagaaaaatccttgcatgtcatttggttcttgttgcagtcttctgtgttcacccctcagaaagcaaaagaatccatctgactttcaataaataccaaattattaaaaaaaaaaaaaaaagaacgtttccacagactagagatccaagaaaaagcagttctgatgaatgattcccagaatcaagtgagtcctcctttagtccaatgagatgatgtcaggaatgttacttccactgctggttatgacccctgtctcactcctgctgctggatgaactaacatgagtactgctttcatgggagctggtggtggtgacagacgtactgcttgctgttaagggtgaggtgagactatccaaaaacataggaggacagtactgctggggatcaactggaataagggaaagaaaatccaaacctggcaaatctgatgacatgcttgatattggcgtatggtggaatggtactgagtagtctgttaatgaaggcggaatagcagcaggatcaaccgaagtcacactgggcacccttacagaagatggctgatacatgagaacccctttggttgggctgctttgtgtttctgacataaagatgcatttccttttggcaggagggtcttcctcttcgtcagaagagctttctattgtaagatcaataacatctactttcttcttgcttgcctcactggctacagtcactgaacaaggcttactgaggacgcttgaactttctatttttgtacacggttggctggatactttcatagcttctttcttcggtctcattggacaccaagaaccatcttcttggaatttgatctcatctacatcagaacagtcattgagaatttccataaaaagcccatctaatattagactttcataggcagcttttttgtcacacacaggacaaatccaggtgggctttttctcattcatttgtagatagagggcagcatcaaaacactgcagatgtgtacaagtcactgcacggcatgggattgtcagcctcatttttcctaaagggcacatcaaggatacccgaaggctagttgtagcaatttcactatcaggatctgcagtaagtttttctttaattagtgctctggaatgatcagggtttctaatacctttcatttttaatctctgtaataacatggctgatgtaagctgccgtacaagatatacagacatagagtaattcttcccaatttctgatgcccaagaaatggaaatttggtttggcacagctgaagataacctaactaaagatgtaatattcaaggggcgtccagggcgcttctgttcaatcccatttttaggcggtggtgcatagccaggcaaaggaaatagcttcccatttacttttatacatagactatttggatagttatcttcttgagggcaacttgtctctgccaggcaaagtctcaactgaacttggactgtataatctctcctaccacctggcaaaaaatccctggatatgcatatctctctaacttgttgaggtgtcaaagcaaaaataaaaaacttctcttgaaatcgctgaatactgctttgaactaaactcgtgggcttgatgagaacatcaaggacatcataaaagggcagattttttaactgcacatcaggatggacaggaggaattgggggagatggctgctgcatctcaaatgtgggcttagtatcttgaagcagcacagaaccaacaggagaggatggtgagtgaggtgtaactgaagtggaaggcaacgagtggattccagccacggccaagtcaggttctacaggtgatgagccaccatccaaactgaaaaccgatgatttgattgtggataaatcagaaagtccttcaagagttcgtggatatcggcgtctatacaattctcggattttaatctgaaccgcagggctgcagccgctcttcaataaatgcagcgccctcatcaggaggtcatgcttgcgtccacttttattccgtccagcaaagcctagtaatacttgtagttcagaaaccctaaaactagaaaccatattcagaatggctaaaatgaaaaacactgataacaccaaatgctggcgaggatgctgagaaactggatcactccatacattgctggtagggatgtaaaatggtacagccactcctcaactcttcgaaatccgccattttataccacccgcgggcgccgccgccgctgccgccgcacccactcccgctgccgccaacgacgctgccgccaccacggccgccgccgcctccagcaccatcctgcactgggcgccgcttaagacgccgcggccgccgccgctacagccgggcccgtcacgt

SEQ ID NO: 13714 - RNA, 8041 nt, Homo sapiens
  source 1..8041: mol_type = other RNA
gctgggattacaggcatgagccaccatgcccagcttaagaattcttgatttttggaaccttgattataagctgcctgatgtctggaaccaaaacttctgtaacactctattccacgtgtacttacaaaacactctaaacatttattaaacagtttgatgaaggccaaaataagaggcatatgctattctacaacacggtaacactcttcgtcacttaaaataattaagctttgagaacacaaaataaagctttttaaaaaagccattcagaaataggaagcagtttgggaaatgattgtgctacgccaatcaagaaaatgttgtacctcaaacatctgaaggtagcaatctgtttttttctttccctgcagctacccttattggaaacataagggaatataaagtgaaaacaggcaatgtttgcctgtttttatagcttttagccttaccacttttcagtttggggatggaatgcctttggctcagtagattctactggctttggggagctcagaaaggccataatggggcctacaggaagaggaaaaagagagctgacctcttaagggcaggccttaggtacaagaggctttttttaaaaagtgacaaaacttttgaactaaagatggaaaacgtagtctgacaaagaatatttgtgcaactttacagtgccagtaaaatcatgggaaaagcttggatagccatacgtaggtgtttctgaaacatgtcagattttatatatatatatatatatatatatatatttttttttttttttttttttttttttagagagtcttgctttgttacccaggctggagtgcagtggcacaatctcggatcactgcaaatcctccgcctcctgggttcaagcgattctcctgcctcggtctcccaagtagctgggactacaggcgcctgccatcacacccacctaatttatgtttttgctagagatggggtttcaccatgttccatgttagccaggctggtctccaactcctgacttcagattatctgcccgccttggcctcccaaagtgctgggattacaggcgtgagcctccatacccggcccatgtcagatatatttaaaactaagaaagcttgggaaaatctctgccaatgatctccatatcagttaaccccgttccatagagtcagaaaggcagagggtcttagtgcagatgcctgcataaagataaaacgttgcatgttcttggaaaatatggctagaccacccttcccataccatctagctgcagtataaattaacatacccatgtggaaaagtggtatgaatcaagaactacaaaagtgttcatatacccttgactagaaattccacctccagtattttatcctaagaaaataatttatacacaaagacattcattgtggcattatgagatataatctaaactgttcaaaataagtaaaggttatatgaaacatggcacatccataacaatggagtaccataaaattaataatagttgacacagttttaatgacatggaataatgcctgtaggttgcggggaaaaaccccaagatataaattacactgagaatgatgaaactaagtaaaaatatgcagaagtagcaaagacaatggcaaggaagatgcaaaaatatcaagtgattttttctggtgacagaatcataggcaattaattgttatacttttctgtattgtctaaattttccacaataagcatgtactactgacataaacagaaaaaacaaacattattcaaccaggcaagcattaaagaatggacattgggtacagctttatttatttcttttaggaattgcaggttcctaacaaagtaggggtgaggggggtgttacaaaccagtcactaggcaggaacattagactccaaaagcagagaaatgcttaattttcttctacctgtttcaccacattcatgtagaactgtagtaaaaaagatggtgaatcaggctgaatcaatctaaataacaacttaaggctcccaaatcacatgaacctaggaccactaaatccaatgtcagacgtgtttaaatggtgcactgctctacatttttctattatgcaaagagctagaaaataatggtagtgtcattatgacattccatgaaaatgaagaaaatctttcaggaaaaattaagaaaataaaaatgtttactaaagaaagaatggtccggctaagtgcttttttttttttttttttttttaaaccaactgaaggccagagaaatgaaaggcatacccgtgaattaaattaatgctttaaaaaaaattgactttacttaaaatacaaacaaacgtcaactaatgaatactttattggcagaaaaaaaagacaacttggctggaaatgctgagtgtcttggactggtctgaaggaagaacatctgaaaggtctgaatgtcaaagtcagaacagtctctggtcaatcctactttgcttaaaatccaacattttacctttcttcaaattcctcaagactaaggaaaacttggttttataccaagaattatgaatcaacctacacttgctatcccttacatcacattttcattctagcttttctgaaacacattaccagataaatgccatataacctaaattcacctcaatgctttcattttgcctttacaattaccttaggacagatgccaagtttttataacttcaggccagaaaatcctcaagtggctcacctaattgtcagaaagtgagtgagtgacaacagacctcaggcacgaaactattttcagcaccaattacactgtggggggttaccagaacaagaaaaggccttcatagttctaagtgaagaaagataaaaacattttattttggccaggcgcggtggctcacgcctgtaaatcccagcactttgggaggccaaggcaggcggatcacctgaggtcgggagttcgagaccagcctgaccaaaatggagaaaccccgtatctactaaaaatacaaaattagctgggcgtggtgatacatgcctgtaatcccagctactcgggaggctgaggcaggagaatcgcttgaaccctgtaggtggaggttgcggtgagccaagatcgcaccattgcactccatcccgggcaacaagagcaagactcagcctcaaaaaaaaaaaaaaaaaaattgattttaggaggctgacaattacagttcatttcctaagatattccagacaatcactggttggctgacagaatctaggtgacagctaagatcacccctctgaaactcccttatatttggttaagcagaaatctgggctagcaaaataaactactagaaagtcagggtctggataagaaacagtgaccacattaaaggctgacggattaataatcatgatgttgccataaggccaaagtcataaagtactaatgctcaagacagataaacaacgtaagccccaatttcaagatgataaacttcaaagtgtattttttaaaatgcaagttgcctgtatgaaataaattaaaaatttatatgtaatttcagtgtaaaacaccaaaaccgaacattaaaactgttcacagaaaatagaaaaaaaaacaaaaaaacaaatcacaattataaaagcacagagatatcagttataagaaccaagtaaataaactaatttctattaatattttcatttactttataaaactttgttgattaaattgggggagtctctgacaatctaaagggtaacaaaataacaaatatacatcatttctttataagtcataccacacaaaccaagttaagttttttctatctgattacagagtcaataaatattgcatctgtatttagagcagcaacataaaactttattagaaagaaatactatatctggaccaaaaaactgcaacatggtttggaaatctaatgactaagaaggtaaaactggcaactatgtgcaactactgctcgtagatttgggtttgtttcccccccaacatctttaaaataagcagcccccacaaagggataatccattgaataaggagacaatgtagccaaagaagggatttgtggaaaaccatatgaatttaaatcaacataaaaagaacacacaaaggccatggaaacttgagaaggtgaaagaaaaaaaaaaaaaaccccaagcaaggacaagtcagctccttggagctgcaccaactcttaagtaggatgtccctattctaacggaaattgatgagtccacacctgggcacttcagtttgagaaatcaattggttggactggccattaaaaaaaggactttgtttttaaggtagataaagcttagagagagaaagctaaacagaaaagtaccaaatccttgtgaactcaaaaatgatttaggaagtcaaatgaagcaaactaaaaaactggatgaaaatgtttctctaagagtaaaacccagttttctctgtgatttaaaatcaaacaaacacactatagaagagaaattttcaaagtgcacccaataaaacctcagaggttccctggagtgtttggggtagcatggattgagacaggaagtgggttcaggcccatctcccccaacccttcttcactttaattcaaacatttctaattctcttttgtcgtttgtagtttcaggtaagatatcattttaaaaaaatgaaaaaaaaaaaaaatctaatgctgtccctttccctaagtttgaaaatcactgctgagactgaaattacattggtgagaaatatgatcatcataaatctaaaacacattttctatgtagtgctaccaaaatacaaagtttcatcaaatatttcactactattctgtaaaataaatgagaaaattaagttgttgggaagaaattaaattttgttattaccacctcccaaaatctgctcttctgctggctccaagatatcaatatttgatagtgtgaacaaatttctaacaaacattccagtcacaccgtaccccaaagacatttcattcaatggctgcatagtttcttttttgagaaggcaagcctcaaatttatagaaaactctagaatgaaaaatgtacaattactaaaaacataataacacactttatgtcagggcagaatctgcatagtgcttttaaacataatcaccaatgaagagtagccaaatcccagaacttcacacagcactcattagcaaacaacgtcaaagtgtaaatgataagcaggaaaaaaaccaagtaacacgaatgccatttttctttgatgcaatcacgaagaaaagtggaaatgcaggacgaaaagtggaatccaagctttggccacgtactgaaacttcattacttcaatgaaacagagcaaatctccatggaaaggactcattcagcaaacattaagttctttccatatattttttttccttcacgtaaggttaaacagaagttgctgtcattctagaatcagtgattacaattttttttttaattagaaaaaaggttacttgaatatttacataattttattgctctttattttaacaaaaacttttttcactgatttgtagactccatccattaacgtatgaaagtgaaatccatctctcaggaagatacagttatggttgaatgtatctgatgctgagagtacagcataattaagaaaaatccttgcatgtcatttggttcttgttgcagtcttctgtgttcacccctcagaaagcaaaagaatccatctgactttcaataaataccaaattattaaaaaaaaaaaaaaaagaacgtttccacagactagagatccaagaaaaagcagttctgatgaatgattcccagaatcaagtgagtcctcctttagtccaatgagatgatgtcaggaatgttacttccactgctggttatgacccctgtctcactcctgctgctggatgaactaacatgagtactgctttcatgggagctggtggtggtgacagacgtactgcttgctgttaagggtgaggtgagactatccaaaaacataggaggacagtactgctggggatcaactggaataagggaaagaaaatccaaacctggcaaatctgatgacatgcttgatattggcgtatggtggaatggtactgagtagtctgttaatgaaggcggaatagcagcaggatcaaccgaagtcacactgggcacccttacagaagatggctgatacatgagaacccctttggttgggctgctttgtgtttctgacataaagatgcatttccttttggcaggagggtcttcctcttcgtcagaagagctttctattgtaagatcaataacatctactttcttcttgcttgcctcactggctacagtcactgaacaaggcttactgaggacgcttgaactttctatttttgtacacggttggctggatactttcatagcttctttcttcggtctcattggacaccaagaaccatcttcttggaatttgatctcatctacatcagaacagtcattgagaatttccataaaaagcccatctaatattagactttcataggcagcttttttgtcacacacaggacaaatccaggtgggctttttctcattcatttgtagatagagggcagcatcaaaacactgcagatgtgtacaagtcactgcacggcatgggattgtcagcctcatttttcctaaagggcacatcaaggatacccgaaggctagttgtagcaatttcactatcaggatctgcagtaagtttttctttaattagtgctctggaatgatcagggtttctaatacctttcatttttaatctctgtaataacatggctgatgtaagctgccgtacaagatatacagacatagagtaattcttcccaatttctgatgcccaagaaatggaaatttggtttggcacagctgaagataacctaactaaagatgtaatattcaaggggcgtccagggcgcttctgttcaatcccatttttaggcggtggtgcatagccaggcaaaggaaatagcttcccatttacttttatacatagactatttggatagttatcttcttgagggcaacttgtctctgccaggcaaagtctcaactgaacttggactgtataatctctcctaccacctggcaaaaaatccctggatatgcatatctctctaacttgttgaggtgtcaaagcaaaaataaaaaacttctcttgaaatcgctgaatactgctttgaactaaactcgtgggcttgatgagaacatcaaggacatcataaaagggcagattttttaactgcacatcaggatggacaggaggaattgggggagatggctgctgcatctcaaatgtgggcttagtatcttgaagcagcacagaaccaacaggagaggatggtgagtgaggtgtaactgaagtggaaggcaacgagtggattccagccacggccaagtcaggttctacaggtgatgagccaccatccaaactgaaaaccgatgatttgattgtggataaatcagaaagtccttcaagagttcgtggatatcggcgtctatacaattctcggattttaatctgaaccgcagggctgcagccgctcttcaataaatgcagcgccctcatcaggaggtcatgcttgcgtccacttttattccgtccagcaaagcctagtaatacttgtagttcagaaaccctaaaactagaaaccatattcagaatggctaaaatgaaaaacactgataacaccaaatgctggcgaggatgctgagaaactggatcactccatacattgctggtagggatgtaaaatggtacagccacttgtgaaactttgaaagcattccctttaaaatcaggaacaagatcaggatgcccccatcacagcttctattcaacattgtactggagatccctcaactcttcgaaatccgccattttataccacccgcgggcgccgccgccgctgccgccgcacccactcccgctgccgccaacgacgctgccgccaccacggccgccgccgcctccagcaccatcctgcactgggcgccgcttaagacgccgcggccgccgccgctacagccgggcccgtcacgt

SEQ ID NO: 13715 - RNA, 7843 nt, Homo sapiens
  source 1..7843: mol_type = other RNA
gctgggattacaggcatgagccaccatgcccagcttaagaattcttgatttttggaaccttgattataagctgcctgatgtctggaaccaaaacttctgtaacactctattccacgtgtacttacaaaacactctaaacatttattaaacagtttgatgaaggccaaaataagaggcatatgctattctacaacacggtaacactcttcgtcacttaaaataattaagctttgagaacacaaaataaagctttttaaaaaagccattcagaaataggaagcagtttgggaaatgattgtgctacgccaatcaagaaaatgttgtacctcaaacatctgaaggtagcaatctgtttttttctttccctgcagctacccttattggaaacataagggaatataaagtgaaaacaggcaatgtttgcctgtttttatagcttttagccttaccacttttcagtttggggatggaatgcctttggctcagtagattctactggctttggggagctcagaaaggccataatggggcctacaggaagaggaaaaagagagctgacctcttaagggcaggccttaggtacaagaggctttttttaaaaagtgacaaaacttttgaactaaagatggaaaacgtagtctgacaaagaatatttgtgcaactttacagtgccagtaaaatcatgggaaaagcttggatagccatacgtaggtgtttctgaaacatgtcagattttatatatatatatatatatatatatatatttttttttttttttttttttttttttagagagtcttgctttgttacccaggctggagtgcagtggcacaatctcggatcactgcaaatcctccgcctcctgggttcaagcgattctcctgcctcggtctcccaagtagctgggactacaggcgcctgccatcacacccacctaatttatgtttttgctagagatggggtttcaccatgttccatgttagccaggctggtctccaactcctgacttcagattatctgcccgccttggcctcccaaagtgctgggattacaggcgtgagcctccatacccggcccatgtcagatatatttaaaactaagaaagcttgggaaaatctctgccaatgatctccatatcagttaaccccgttccatagagtcagaaaggcagagggtcttagtgcagatgcctgcataaagataaaacgttgcatgttcttggaaaatatggctagaccacccttcccataccatctagctgcagtataaattaacatacccatgtggaaaagtggtatgaatcaagaactacaaaagtgttcatatacccttgactagaaattccacctccagtattttatcctaagaaaataatttatacacaaagacattcattgtggcattatgagatataatctaaactgttcaaaataagtaaaggttatatgaaacatggcacatccataacaatggagtaccataaaattaataatagttgacacagttttaatgacatggaataatgcctgtaggttgcggggaaaaaccccaagatataaattacactgagaatgatgaaactaagtaaaaatatgcagaagtagcaaagacaatggcaaggaagatgcaaaaatatcaagtgattttttctggtgacagaatcataggcaattaattgttatacttttctgtattgtctaaattttccacaataagcatgtactactgacataaacagaaaaaacaaacattattcaaccaggcaagcattaaagaatggacattgggtacagctttatttatttcttttaggaattgcaggttcctaacaaagtaggggtgaggggggtgttacaaaccagtcactaggcaggaacattagactccaaaagcagagaaatgcttaattttcttctacctgtttcaccacattcatgtagaactgtagtaaaaaagatggtgaatcaggctgaatcaatctaaataacaacttaaggctcccaaatcacatgaacctaggaccactaaatccaatgtcagacgtgtttaaatggtgcactgctctacatttttctattatgcaaagagctagaaaataatggtagtgtcattatgacattccatgaaaatgaagaaaatctttcaggaaaaattaagaaaataaaaatgtttactaaagaaagaatggtccggctaagtgcttttttttttttttttttttttaaaccaactgaaggccagagaaatgaaaggcatacccgtgaattaaattaatgctttaaaaaaaattgactttacttaaaatacaaacaaacgtcaactaatgaatactttattggcagaaaaaaaagacaacttggctggaaatgctgagtgtcttggactggtctgaaggaagaacatctgaaaggtctgaatgtcaaagtcagaacagtctctggtcaatcctactttgcttaaaatccaacattttacctttcttcaaattcctcaagactaaggaaaacttggttttataccaagaattatgaatcaacctacacttgctatcccttacatcacattttcattctagcttttctgaaacacattaccagataaatgccatataacctaaattcacctcaatgctttcattttgcctttacaattaccttaggacagatgccaagtttttataacttcaggccagaaaatcctcaagtggctcacctaattgtcagaaagtgagtgagtgacaacagacctcaggcacgaaactattttcagcaccaattacactgtggggggttaccagaacaagaaaaggccttcatagttctaagtgaagaaagataaaaacattttattttggccaggcgcggtggctcacgcctgtaaatcccagcactttgggaggccaaggcaggcggatcacctgaggtcgggagttcgagaccagcctgaccaaaatggagaaaccccgtatctactaaaaatacaaaattagctgggcgtggtgatacatgcctgtaatcccagctactcgggaggctgaggcaggagaatcgcttgaaccctgtaggtggaggttgcggtgagccaagatcgcaccattgcactccatcccgggcaacaagagcaagactcagcctcaaaaaaaaaaaaaaaaaaattgattttaggaggctgacaattacagttcatttcctaagatattccagacaatcactggttggctgacagaatctaggtgacagctaagatcacccctctgaaactcccttatatttggttaagcagaaatctgggctagcaaaataaactactagaaagtcagggtctggataagaaacagtgaccacattaaaggctgacggattaataatcatgatgttgccataaggccaaagtcataaagtactaatgctcaagacagataaacaacgtaagccccaatttcaagatgataaacttcaaagtgtattttttaaaatgcaagttgcctgtatgaaataaattaaaaatttatatgtaatttcagtgtaaaacaccaaaaccgaacattaaaactgttcacagaaaatagaaaaaaaaacaaaaaaacaaatcacaattataaaagcacagagatatcagttataagaaccaagtaaataaactaatttctattaatattttcatttactttataaaactttgttgattaaattgggggagtctctgacaatctaaagggtaacaaaataacaaatatacatcatttctttataagtcataccacacaaaccaagttaagttttttctatctgattacagagtcaataaatattgcatctgtatttagagcagcaacataaaactttattagaaagaaatactatatctggaccaaaaaactgcaacatggtttggaaatctaatgactaagaaggtaaaactggcaactatgtgcaactactgctcgtagatttgggtttgtttcccccccaacatctttaaaataagcagcccccacaaagggataatccattgaataaggagacaatgtagccaaagaagggatttgtggaaaaccatatgaatttaaatcaacataaaaagaacacacaaaggccatggaaacttgagaaggtgaaagaaaaaaaaaaaaaaccccaagcaaggacaagtcagctccttggagctgcaccaactcttaagtaggatgtccctattctaacggaaattgatgagtccacacctgggcacttcagtttgagaaatcaattggttggactggccattaaaaaaaggactttgtttttaaggtagataaagcttagagagagaaagctaaacagaaaagtaccaaatccttgtgaactcaaaaatgatttaggaagtcaaatgaagcaaactaaaaaactggatgaaaatgtttctctaagagtaaaacccagttttctctgtgatttaaaatcaaacaaacacactatagaagagaaattttcaaagtgcacccaataaaacctcagaggttccctggagtgtttggggtagcatggattgagacaggaagtgggttcaggcccatctcccccaacccttcttcactttaattcaaacatttctaattctcttttgtcgtttgtagtttcaggtaagatatcattttaaaaaaatgaaaaaaaaaaaaaatctaatgctgtccctttccctaagtttgaaaatcactgctgagactgaaattacattggtgagaaatatgatcatcataaatctaaaacacattttctatgtagtgctaccaaaatacaaagtttcatcaaatatttcactactattctgtaaaataaatgagaaaattaagttgttgggaagaaattaaattttgttattaccacctcccaaaatctgctcttctgctggctccaagatatcaatatttgatagtgtgaacaaatttctaacaaacattccagtcacaccgtaccccaaagacatttcattcaatggctgcatagtttcttttttgagaaggcaagcctcaaatttatagaaaactctagaatgaaaaatgtacaattactaaaaacataataacacactttatgtcagggcagaatctgcatagtgcttttaaacataatcaccaatgaagagtagccaaatcccagaacttcacacagcactcattagcaaacaacgtcaaagtgtaaatgataagcaggaaaaaaaccaagtaacacgaatgccatttttctttgatgcaatcacgaagaaaagtggaaatgcaggacgaaaagtggaatccaagctttggccacgtactgaaacttcattacttcaatgaaacagagcaaatctccatggaaaggactcattcagcaaacattaagttctttccatatattttttttccttcacgtaaggttaaacagaagttgctgtcattctagaatcagtgattacaattttttttttaattagaaaaaaggttacttgaatatttacataattttattgctctttattttaacaaaaacttttttcactgatttgtagactccatccattaacgtatgaaagtgaaatccatctctcaggaagatacagttatggttgaatgtatctgatgctgagagtacagcataattaagaaaaatccttgcatgtcatttggttcttgttgcagtcttctgtgttcacccctcagaaagcaaaagaatccatctgactttcaataaataccaaattattaaaaaaaaaaaaaaaagaacgtttccacagactagagatccaagaaaaagcagttctgatgaatgattcccagaatcaagtgagtcctcctttagtccaatgagatgatgtcaggaatgttacttccactgctggttatgacccctgtctcactcctgctgctggatgaactaacatgagtactgctttcatgggagctggtggtggtgacagacgtactgcttgctgttaagggtgaggtgagactatccaaaaacataggaggacagtactgctggggatcaactggaataagggaaagaaaatccaaacctggcaaatctgatgacatgcttgatattggcgtatggtggaatggtactgagtagtctgttaatgaaggcggaatagcagcaggatcaaccgaagtcacactgggcacccttacagaagatggctgatacatgagaacccctttggttgggctgctttgtgtttctgacataaagatgcatttccttttggcaggagggtcttcctcttcgtcagaagagctttctattgtaagatcaataacatctactttcttcttgcttgcctcactggctacagtcactgaacaaggcttactgaggacgcttgaactttctatttttgtacacggttggctggatactttcatagcttctttcttcggtctcattggacaccaagaaccatcttcttggaatttgatctcatctacatcagaacagtcattgagaatttccataaaaagcccatctaatattagactttcataggcagcttttttgtcacacacaggacaaatccaggtgggctttttctcattcatttgtagatagagggcagcatcaaaacactgcagatgtgtacaagtcactgcacggcatgggattgtcagcctcatttttcctaaagggcacatcaaggatacccgaaggctagttgtagcaatttcactatcaggatctgcagtaagtttttctttaattagtgctctggaatgatcagggtttctaatacctttcatttttaatctctgtaataacatggctgatgtaagctgccgtacaagatatacagacatagagtaattcttcccaatttctgatgcccaagaaatggaaatttggtttggcacagctgaagataacctaactaaagatgtaatattcaaggggcgtccagggcgcttctgttcaatcccatttttaggcggtggtgcatagccaggcaaaggaaatagcttcccatttacttttatacatagactatttggatagttatcttcttgagggcaacttgtctctgccaggcaaagtctcaactgaacttggactgtataatctctcctaccacctggcaaaaaatccctggatatgcatatctctctaacttgttgaggtgtcaaagcaaaaataaaaaacttctcttgaaatcgctgaatactgctttgaactaaactcgtgggcttgatgagaacatcaaggacatcataaaagggcagattttttaactgcacatcaggatggacaggaggaattgggggagatggctgctgcatctcaaatgtgggcttagtatcttgaagcagcacagaaccaacaggagaggatggtgagtgaggtgtaactgaagtggaaggcaacgagtggattccagccacggccaagtcaggttctacaggtgatgagccaccatccaaactgaaaaccgatgatttgattgtggataaatcagaaagtccttcaagagttcgtggatatcggcgtctatacaattctcggattttaatctgaaccgcagggctgcagccgctcttcaataaatgcagcgccctcatcaggaggtcatgcttgcgtccacttttattccgtccagcaaagcctagtaatacttgtagttcagaaaccctaaaactagaaaccatattcctcaactcttcgaaatccgccattttataccacccgcgggcgccgccgccgctgccgccgcacccactcccgctgccgccaacgacgctgccgccaccacggccgccgccgcctccagcaccatcctgcactgggcgccgcttaagacgccgcggccgccgccgctacagccgggcccgtcacgt

SEQ ID NO: 13716 - RNA, 8142 nt, Homo sapiens
  source 1..8142: mol_type = other RNA
gctgggattacaggcatgagccaccatgcccagcttaagaattcttgatttttggaaccttgattataagctgcctgatgtctggaaccaaaacttctgtaacactctattccacgtgtacttacaaaacactctaaacatttattaaacagtttgatgaaggccaaaataagaggcatatgctattctacaacacggtaacactcttcgtcacttaaaataattaagctttgagaacacaaaataaagctttttaaaaaagccattcagaaataggaagcagtttgggaaatgattgtgctacgccaatcaagaaaatgttgtacctcaaacatctgaaggtagcaatctgtttttttctttccctgcagctacccttattggaaacataagggaatataaagtgaaaacaggcaatgtttgcctgtttttatagcttttagccttaccacttttcagtttggggatggaatgcctttggctcagtagattctactggctttggggagctcagaaaggccataatggggcctacaggaagaggaaaaagagagctgacctcttaagggcaggccttaggtacaagaggctttttttaaaaagtgacaaaacttttgaactaaagatggaaaacgtagtctgacaaagaatatttgtgcaactttacagtgccagtaaaatcatgggaaaagcttggatagccatacgtaggtgtttctgaaacatgtcagattttatatatatatatatatatatatatatatttttttttttttttttttttttttttagagagtcttgctttgttacccaggctggagtgcagtggcacaatctcggatcactgcaaatcctccgcctcctgggttcaagcgattctcctgcctcggtctcccaagtagctgggactacaggcgcctgccatcacacccacctaatttatgtttttgctagagatggggtttcaccatgttccatgttagccaggctggtctccaactcctgacttcagattatctgcccgccttggcctcccaaagtgctgggattacaggcgtgagcctccatacccggcccatgtcagatatatttaaaactaagaaagcttgggaaaatctctgccaatgatctccatatcagttaaccccgttccatagagtcagaaaggcagagggtcttagtgcagatgcctgcataaagataaaacgttgcatgttcttggaaaatatggctagaccacccttcccataccatctagctgcagtataaattaacatacccatgtggaaaagtggtatgaatcaagaactacaaaagtgttcatatacccttgactagaaattccacctccagtattttatcctaagaaaataatttatacacaaagacattcattgtggcattatgagatataatctaaactgttcaaaataagtaaaggttatatgaaacatggcacatccataacaatggagtaccataaaattaataatagttgacacagttttaatgacatggaataatgcctgtaggttgcggggaaaaaccccaagatataaattacactgagaatgatgaaactaagtaaaaatatgcagaagtagcaaagacaatggcaaggaagatgcaaaaatatcaagtgattttttctggtgacagaatcataggcaattaattgttatacttttctgtattgtctaaattttccacaataagcatgtactactgacataaacagaaaaaacaaacattattcaaccaggcaagcattaaagaatggacattgggtacagctttatttatttcttttaggaattgcaggttcctaacaaagtaggggtgaggggggtgttacaaaccagtcactaggcaggaacattagactccaaaagcagagaaatgcttaattttcttctacctgtttcaccacattcatgtagaactgtagtaaaaaagatggtgaatcaggctgaatcaatctaaataacaacttaaggctcccaaatcacatgaacctaggaccactaaatccaatgtcagacgtgtttaaatggtgcactgctctacatttttctattatgcaaagagctagaaaataatggtagtgtcattatgacattccatgaaaatgaagaaaatctttcaggaaaaattaagaaaataaaaatgtttactaaagaaagaatggtccggctaagtgcttttttttttttttttttttttaaaccaactgaaggccagagaaatgaaaggcatacccgtgaattaaattaatgctttaaaaaaaattgactttacttaaaatacaaacaaacgtcaactaatgaatactttattggcagaaaaaaaagacaacttggctggaaatgctgagtgtcttggactggtctgaaggaagaacatctgaaaggtctgaatgtcaaagtcagaacagtctctggtcaatcctactttgcttaaaatccaacattttacctttcttcaaattcctcaagactaaggaaaacttggttttataccaagaattatgaatcaacctacacttgctatcccttacatcacattttcattctagcttttctgaaacacattaccagataaatgccatataacctaaattcacctcaatgctttcattttgcctttacaattaccttaggacagatgccaagtttttataacttcaggccagaaaatcctcaagtggctcacctaattgtcagaaagtgagtgagtgacaacagacctcaggcacgaaactattttcagcaccaattacactgtggggggttaccagaacaagaaaaggccttcatagttctaagtgaagaaagataaaaacattttattttggccaggcgcggtggctcacgcctgtaaatcccagcactttgggaggccaaggcaggcggatcacctgaggtcgggagttcgagaccagcctgaccaaaatggagaaaccccgtatctactaaaaatacaaaattagctgggcgtggtgatacatgcctgtaatcccagctactcgggaggctgaggcaggagaatcgcttgaaccctgtaggtggaggttgcggtgagccaagatcgcaccattgcactccatcccgggcaacaagagcaagactcagcctcaaaaaaaaaaaaaaaaaaattgattttaggaggctgacaattacagttcatttcctaagatattccagacaatcactggttggctgacagaatctaggtgacagctaagatcacccctctgaaactcccttatatttggttaagcagaaatctgggctagcaaaataaactactagaaagtcagggtctggataagaaacagtgaccacattaaaggctgacggattaataatcatgatgttgccataaggccaaagtcataaagtactaatgctcaagacagataaacaacgtaagccccaatttcaagatgataaacttcaaagtgtattttttaaaatgcaagttgcctgtatgaaataaattaaaaatttatatgtaatttcagtgtaaaacaccaaaaccgaacattaaaactgttcacagaaaatagaaaaaaaaacaaaaaaacaaatcacaattataaaagcacagagatatcagttataagaaccaagtaaataaactaatttctattaatattttcatttactttataaaactttgttgattaaattgggggagtctctgacaatctaaagggtaacaaaataacaaatatacatcatttctttataagtcataccacacaaaccaagttaagttttttctatctgattacagagtcaataaatattgcatctgtatttagagcagcaacataaaactttattagaaagaaatactatatctggaccaaaaaactgcaacatggtttggaaatctaatgactaagaaggtaaaactggcaactatgtgcaactactgctcgtagatttgggtttgtttcccccccaacatctttaaaataagcagcccccacaaagggataatccattgaataaggagacaatgtagccaaagaagggatttgtggaaaaccatatgaatttaaatcaacataaaaagaacacacaaaggccatggaaacttgagaaggtgaaagaaaaaaaaaaaaaaccccaagcaaggacaagtcagctccttggagctgcaccaactcttaagtaggatgtccctattctaacggaaattgatgagtccacacctgggcacttcagtttgagaaatcaattggttggactggccattaaaaaaaggactttgtttttaaggtagataaagcttagagagagaaagctaaacagaaaagtaccaaatccttgtgaactcaaaaatgatttaggaagtcaaatgaagcaaactaaaaaactggatgaaaatgtttctctaagagtaaaacccagttttctctgtgatttaaaatcaaacaaacacactatagaagagaaattttcaaagtgcacccaataaaacctcagaggttccctggagtgtttggggtagcatggattgagacaggaagtgggttcaggcccatctcccccaacccttcttcactttaattcaaacatttctaattctcttttgtcgtttgtagtttcaggtaagatatcattttaaaaaaatgaaaaaaaaaaaaaatctaatgctgtccctttccctaagtttgaaaatcactgctgagactgaaattacattggtgagaaatatgatcatcataaatctaaaacacattttctatgtagtgctaccaaaatacaaagtttcatcaaatatttcactactattctgtaaaataaatgagaaaattaagttgttgggaagaaattaaattttgttattaccacctcccaaaatctgctcttctgctggctccaagatatcaatatttgatagtgtgaacaaatttctaacaaacattccagtcacaccgtaccccaaagacatttcattcaatggctgcatagtttcttttttgagaaggcaagcctcaaatttatagaaaactctagaatgaaaaatgtacaattactaaaaacataataacacactttatgtcagggcagaatctgcatagtgcttttaaacataatcaccaatgaagagtagccaaatcccagaacttcacacagcactcattagcaaacaacgtcaaagtgtaaatgataagcaggaaaaaaaccaagtaacacgaatgccatttttctttgatgcaatcacgaagaaaagtggaaatgcaggacgaaaagtggaatccaagctttggccacgtactgaaacttcattacttcaatgaaacagagcaaatctccatggaaaggactcattcagcaaacattaagttctttccatatattttttttccttcacgtaaggttaaacagaagttgctgtcattctagaatcagtgattacaattttttttttaattagaaaaaaggttacttgaatatttacataattttattgctctttattttaacaaaaacttttttcactgatttgtagactccatccattaacgtatgaaagtgaaatccatctctcaggaagatacagttatggttgaatgtatctgatgctgagagtacagcataattaagaaaaatccttgcatgtcatttggttcttgttgcagtcttctgtgttcacccctcagaaagcaaaagaatccatctgactttcaataaataccaaattattaaaaaaaaaaaaaaaagaacgtttccacagactagagatccaagaaaaagcagttctgatgaatgattcccagaatcaagtgagtcctcctttagtccaatgagatgatgtcaggaatgttacttccactgctggttatgacccctgtctcactcctgctgctggatgaactaacatgagtactgctttcatgggagctggtggtggtgacagacgtactgcttgctgttaagggtgaggtgagactatccaaaaacataggaggacagtactgctggggatcaactggaataagggaaagaaaatccaaacctggcaaatctgatgacatgcttgatattggcgtatggtggaatggtactgagtagtctgttaatgaaggcggaatagcagcaggatcaaccgaagtcacactgggcacccttacagaagatggctgatacatgagaacccctttggttgggctgctttgtgtttctgacataaagatgcatttccttttggcaggagggtcttcctcttcgtcagaagagctttctattgtaagatcaataacatctactttcttcttgcttgcctcactggctacagtcactgaacaaggcttactgaggacgcttgaactttctatttttgtacacggttggctggatactttcatagcttctttcttcggtctcattggacaccaagaaccatcttcttggaatttgatctcatctacatcagaacagtcattgagaatttccataaaaagcccatctaatattagactttcataggcagcttttttgtcacacacaggacaaatccaggtgggctttttctcattcatttgtagatagagggcagcatcaaaacactgcagatgtgtacaagtcactgcacggcatgggattgtcagcctcatttttcctaaagggcacatcaaggatacccgaaggctagttgtagcaatttcactatcaggatctgcagtaagtttttctttaattagtgctctggaatgatcagggtttctaatacctttcatttttaatctctgtaataacatggctgatgtaagctgccgtacaagatatacagacatagagtaattcttcccaatttctgatgcccaagaaatggaaatttggtttggcacagctgaagataacctaactaaagatgtaatattcaaggggcgtccagggcgcttctgttcaatcccatttttaggcggtggtgcatagccaggcaaaggaaatagcttcccatttacttttatacatagactatttggatagttatcttcttgagggcaacttgtctctgccaggcaaagtctcaactgaacttggactgtataatctctcctaccacctggcaaaaaatccctggatatgcatatctctctaacttgttgaggtgtcaaagcaaaaataaaaaacttctcttgaaatcgctgaatactgctttgaactaaactcgtgggcttgatgagaacatcaaggacatcataaaagggcagattttttaactgcacatcaggatggacaggaggaattgggggagatggctgctgcatctcaaatgtgggcttagtatcttgaagcagcacagaaccaacaggagaggatggtgagtgaggtgtaactgaagtggaaggcaacgagtggattccagccacggccaagtcaggttctacaggtgatgagccaccatccaaactgaaaaccgatgatttgattgtggataaatcagaaagtccttcaagagttcgtggatatcggcgtctatacaattctcggattttaatctgaaccgcagggctgcagccgctcttcaataaatgcagcgccctcatcaggaggtcatgcttgcgtccacttttattccgtccagcaaagcctagtaatacttgtagttcagaaaccctaaaactagaaaccatattctaagcttgactctcagaggaatttctaggaggtctcatatctcatatttccagtgataacattatttggcaaaggatgttaatgcaactggctctatgggcagaatggctaaaatgaaaaacactgataacaccaaatgctggcgaggatgctgagaaactggatcactccatacattgctggtagggatgtaaaatggtacagccacttgtgaaactttgaaagcattccctttaaaatcaggaacaagatcaggatgcccccatcacagcttctattcaacattgtactggagatccctcaactcttcgaaatccgccattttataccacccgcgggcgccgccgccgctgccgccgcacccactcccgctgccgccaacgacgctgccgccaccacggccgccgccgcctccagcaccatcctgcactgggcgccgcttaagacgccgcggccgccgccgctacagccgggcccgtcacgt

SEQ ID NO: 13717 - RNA, 8119 nt, Homo sapiens
  source 1..8119: mol_type = other RNA
gctgggattacaggcatgagccaccatgcccagcttaagaattcttgatttttggaaccttgattataagctgcctgatgtctggaaccaaaacttctgtaacactctattccacgtgtacttacaaaacactctaaacatttattaaacagtttgatgaaggccaaaataagaggcatatgctattctacaacacggtaacactcttcgtcacttaaaataattaagctttgagaacacaaaataaagctttttaaaaaagccattcagaaataggaagcagtttgggaaatgattgtgctacgccaatcaagaaaatgttgtacctcaaacatctgaaggtagcaatctgtttttttctttccctgcagctacccttattggaaacataagggaatataaagtgaaaacaggcaatgtttgcctgtttttatagcttttagccttaccacttttcagtttggggatggaatgcctttggctcagtagattctactggctttggggagctcagaaaggccataatggggcctacaggaagaggaaaaagagagctgacctcttaagggcaggccttaggtacaagaggctttttttaaaaagtgacaaaacttttgaactaaagatggaaaacgtagtctgacaaagaatatttgtgcaactttacagtgccagtaaaatcatgggaaaagcttggatagccatacgtaggtgtttctgaaacatgtcagattttatatatatatatatatatatatatatatttttttttttttttttttttttttttagagagtcttgctttgttacccaggctggagtgcagtggcacaatctcggatcactgcaaatcctccgcctcctgggttcaagcgattctcctgcctcggtctcccaagtagctgggactacaggcgcctgccatcacacccacctaatttatgtttttgctagagatggggtttcaccatgttccatgttagccaggctggtctccaactcctgacttcagattatctgcccgccttggcctcccaaagtgctgggattacaggcgtgagcctccatacccggcccatgtcagatatatttaaaactaagaaagcttgggaaaatctctgccaatgatctccatatcagttaaccccgttccatagagtcagaaaggcagagggtcttagtgcagatgcctgcataaagataaaacgttgcatgttcttggaaaatatggctagaccacccttcccataccatctagctgcagtataaattaacatacccatgtggaaaagtggtatgaatcaagaactacaaaagtgttcatatacccttgactagaaattccacctccagtattttatcctaagaaaataatttatacacaaagacattcattgtggcattatgagatataatctaaactgttcaaaataagtaaaggttatatgaaacatggcacatccataacaatggagtaccataaaattaataatagttgacacagttttaatgacatggaataatgcctgtaggttgcggggaaaaaccccaagatataaattacactgagaatgatgaaactaagtaaaaatatgcagaagtagcaaagacaatggcaaggaagatgcaaaaatatcaagtgattttttctggtgacagaatcataggcaattaattgttatacttttctgtattgtctaaattttccacaataagcatgtactactgacataaacagaaaaaacaaacattattcaaccaggcaagcattaaagaatggacattgggtacagctttatttatttcttttaggaattgcaggttcctaacaaagtaggggtgaggggggtgttacaaaccagtcactaggcaggaacattagactccaaaagcagagaaatgcttaattttcttctacctgtttcaccacattcatgtagaactgtagtaaaaaagatggtgaatcaggctgaatcaatctaaataacaacttaaggctcccaaatcacatgaacctaggaccactaaatccaatgtcagacgtgtttaaatggtgcactgctctacatttttctattatgcaaagagctagaaaataatggtagtgtcattatgacattccatgaaaatgaagaaaatctttcaggaaaaattaagaaaataaaaatgtttactaaagaaagaatggtccggctaagtgcttttttttttttttttttttttaaaccaactgaaggccagagaaatgaaaggcatacccgtgaattaaattaatgctttaaaaaaaattgactttacttaaaatacaaacaaacgtcaactaatgaatactttattggcagaaaaaaaagacaacttggctggaaatgctgagtgtcttggactggtctgaaggaagaacatctgaaaggtctgaatgtcaaagtcagaacagtctctggtcaatcctactttgcttaaaatccaacattttacctttcttcaaattcctcaagactaaggaaaacttggttttataccaagaattatgaatcaacctacacttgctatcccttacatcacattttcattctagcttttctgaaacacattaccagataaatgccatataacctaaattcacctcaatgctttcattttgcctttacaattaccttaggacagatgccaagtttttataacttcaggccagaaaatcctcaagtggctcacctaattgtcagaaagtgagtgagtgacaacagacctcaggcacgaaactattttcagcaccaattacactgtggggggttaccagaacaagaaaaggccttcatagttctaagtgaagaaagataaaaacattttattttggccaggcgcggtggctcacgcctgtaaatcccagcactttgggaggccaaggcaggcggatcacctgaggtcgggagttcgagaccagcctgaccaaaatggagaaaccccgtatctactaaaaatacaaaattagctgggcgtggtgatacatgcctgtaatcccagctactcgggaggctgaggcaggagaatcgcttgaaccctgtaggtggaggttgcggtgagccaagatcgcaccattgcactccatcccgggcaacaagagcaagactcagcctcaaaaaaaaaaaaaaaaaaattgattttaggaggctgacaattacagttcatttcctaagatattccagacaatcactggttggctgacagaatctaggtgacagctaagatcacccctctgaaactcccttatatttggttaagcagaaatctgggctagcaaaataaactactagaaagtcagggtctggataagaaacagtgaccacattaaaggctgacggattaataatcatgatgttgccataaggccaaagtcataaagtactaatgctcaagacagataaacaacgtaagccccaatttcaagatgataaacttcaaagtgtattttttaaaatgcaagttgcctgtatgaaataaattaaaaatttatatgtaatttcagtgtaaaacaccaaaaccgaacattaaaactgttcacagaaaatagaaaaaaaaacaaaaaaacaaatcacaattataaaagcacagagatatcagttataagaaccaagtaaataaactaatttctattaatattttcatttactttataaaactttgttgattaaattgggggagtctctgacaatctaaagggtaacaaaataacaaatatacatcatttctttataagtcataccacacaaaccaagttaagttttttctatctgattacagagtcaataaatattgcatctgtatttagagcagcaacataaaactttattagaaagaaatactatatctggaccaaaaaactgcaacatggtttggaaatctaatgactaagaaggtaaaactggcaactatgtgcaactactgctcgtagatttgggtttgtttcccccccaacatctttaaaataagcagcccccacaaagggataatccattgaataaggagacaatgtagccaaagaagggatttgtggaaaaccatatgaatttaaatcaacataaaaagaacacacaaaggccatggaaacttgagaaggtgaaagaaaaaaaaaaaaaaccccaagcaaggacaagtcagctccttggagctgcaccaactcttaagtaggatgtccctattctaacggaaattgatgagtccacacctgggcacttcagtttgagaaatcaattggttggactggccattaaaaaaaggactttgtttttaaggtagataaagcttagagagagaaagctaaacagaaaagtaccaaatccttgtgaactcaaaaatgatttaggaagtcaaatgaagcaaactaaaaaactggatgaaaatgtttctctaagagtaaaacccagttttctctgtgatttaaaatcaaacaaacacactatagaagagaaattttcaaagtgcacccaataaaacctcagaggttccctggagtgtttggggtagcatggattgagacaggaagtgggttcaggcccatctcccccaacccttcttcactttaattcaaacatttctaattctcttttgtcgtttgtagtttcaggtaagatatcattttaaaaaaatgaaaaaaaaaaaaaatctaatgctgtccctttccctaagtttgaaaatcactgctgagactgaaattacattggtgagaaatatgatcatcataaatctaaaacacattttctatgtagtgctaccaaaatacaaagtttcatcaaatatttcactactattctgtaaaataaatgagaaaattaagttgttgggaagaaattaaattttgttattaccacctcccaaaatctgctcttctgctggctccaagatatcaatatttgatagtgtgaacaaatttctaacaaacattccagtcacaccgtaccccaaagacatttcattcaatggctgcatagtttcttttttgagaaggcaagcctcaaatttatagaaaactctagaatgaaaaatgtacaattactaaaaacataataacacactttatgtcagggcagaatctgcatagtgcttttaaacataatcaccaatgaagagtagccaaatcccagaacttcacacagcactcattagcaaacaacgtcaaagtgtaaatgataagcaggaaaaaaaccaagtaacacgaatgccatttttctttgatgcaatcacgaagaaaagtggaaatgcaggacgaaaagtggaatccaagctttggccacgtactgaaacttcattacttcaatgaaacagagcaaatctccatggaaaggactcattcagcaaacattaagttctttccatatattttttttccttcacgtaaggttaaacagaagttgctgtcattctagaatcagtgattacaattttttttttaattagaaaaaaggttacttgaatatttacataattttattgctctttattttaacaaaaacttttttcactgatttgtagactccatccattaacgtatgaaagtgaaatccatctctcaggaagatacagttatggttgaatgtatctgatgctgagagtacagcataattaagaaaaatccttgcatgtcatttggttcttgttgcagtcttctgtgttcacccctcagaaagcaaaagaatccatctgactttcaataaataccaaattattaaaaaaaaaaaaaaaagaacgtttccacagactagagatccaagaaaaagcagttctgatgaatgattcccagaatcaagtgagtcctcctttagtccaatgagatgatgtcaggaatgttacttccactgctggttatgacccctgtctcactcctgctgctggatgaactaacatgagtactgctttcatgggagctggtggtggtgacagacgtactgcttgctgttaagggtgaggtgagactatccaaaaacataggaggacagtactggggatcaactggaataagggaaagaaaatccaaacctgacaatatggcactagcaataataaggcagtcatatttttccttgaaataagctgttttccactccataaatacaaattatttgttttattttgtattcactgttgcacagtatcagaagatgttccaagcttcagttcattattaatatcatttcttctttgttctcctggcaaatctgatgacatgcttgatattggcgtatggtggaatggtactgagtagtctgttaatgaaggcggaatagcagcaggatcaaccgaagtcacactgggcacccttacagaagatggctgatacatgagaacccctttggttgggctgctttgtgtttctgacataaagatgcatttccttttggcaggagggtcttcctcttcgtcagaagagctttctattgtaagatcaataacatctactttcttcttgcttgcctcactggctacagtcactgaacaaggcttactgaggacgcttgaactttctatttttgtacacggttggctggatactttcatagcttctttcttcggtctcattggacaccaagaaccatcttcttggaatttgatctcatctacatcagaacagtcattgagaatttccataaaaagcccatctaatattagactttcataggcagcttttttgtcacacacaggacaaatccaggtgggctttttctcattcatttgtagatagagggcagcatcaaaacactgcagatgtgtacaagtcactgcacggcatgggattgtcagcctcatttttcctaaagggcacatcaaggatacccgaaggctagttgtagcaatttcactatcaggatctgcagtaagtttttctttaattagtgctctggaatgatcagggtttctaatacctttcatttttaatctctgtaataacatggctgatgtaagctgccgtacaagatatacagacatagagtaattcttcccaatttctgatgcccaagaaatggaaatttggtttggcacagctgaagataacctaactaaagatgtaatattcaaggggcgtccagggcgcttctgttcaatcccatttttaggcggtggtgcatagccaggcaaaggaaatagcttcccatttacttttatacatagactatttggatagttatcttcttgagggcaacttgtctctgccaggcaaagtctcaactgaacttggactgtataatctctcctaccacctggcaaaaaatccctggatatgcatatctctctaacttgttgaggtgtcaaagcaaaaataaaaaacttctcttgaaatcgctgaatactgctttgaactaaactcgtgggcttgatgagaacatcaaggacatcataaaagggcagattttttaactgcacatcaggatggacaggaggaattgggggagatggctgctgcatctcaaatgtgggcttagtatcttgaagcagcacagaaccaacaggagaggatggtgagtgaggtgtaactgaagtggaaggcaacgagtggattccagccacggccaagtcaggttctacaggtgatgagccaccatccaaactgaaaaccgatgatttgattgtggataaatcagaaagtccttcaagagttcgtggatatcggcgtctatacaattctcggattttaatctgaaccgcagggctgcagccgctcttcaataaatgcagcgccctcatcaggaggtcatgcttgcgtccacttttattccgtccagcaaagcctagtaatacttgtagttcagaaaccctaaaactagaaaccatattcagaatggctaaaatgaaaaacactgataacaccaaatgctggcgaggatgctgagaaactggatcactccatacattgctggtagggatgtaaaatggtacagccactcctcaactcttcgaaatccgccattttataccacccgcgggcgccgccgccgctgccgccgcacccactcccgctgccgccaacgacgctgccgccaccacggccgccgccgcctccagcaccatcctgcactgggcgccgcttaagacgccgcggccgccgccgctacagccgggcccgtcacgt

SEQ ID NO: 13718 - RNA, 8010 nt, Homo sapiens
  source 1..8010: mol_type = other RNA
gctgggattacaggcatgagccaccatgcccagcttaagaattcttgatttttggaaccttgattataagctgcctgatgtctggaaccaaaacttctgtaacactctattccacgtgtacttacaaaacactctaaacatttattaaacagtttgatgaaggccaaaataagaggcatatgctattctacaacacggtaacactcttcgtcacttaaaataattaagctttgagaacacaaaataaagctttttaaaaaagccattcagaaataggaagcagtttgggaaatgattgtgctacgccaatcaagaaaatgttgtacctcaaacatctgaaggtagcaatctgtttttttctttccctgcagctacccttattggaaacataagggaatataaagtgaaaacaggcaatgtttgcctgtttttatagcttttagccttaccacttttcagtttggggatggaatgcctttggctcagtagattctactggctttggggagctcagaaaggccataatggggcctacaggaagaggaaaaagagagctgacctcttaagggcaggccttaggtacaagaggctttttttaaaaagtgacaaaacttttgaactaaagatggaaaacgtagtctgacaaagaatatttgtgcaactttacagtgccagtaaaatcatgggaaaagcttggatagccatacgtaggtgtttctgaaacatgtcagattttatatatatatatatatatatatatatatttttttttttttttttttttttttttagagagtcttgctttgttacccaggctggagtgcagtggcacaatctcggatcactgcaaatcctccgcctcctgggttcaagcgattctcctgcctcggtctcccaagtagctgggactacaggcgcctgccatcacacccacctaatttatgtttttgctagagatggggtttcaccatgttccatgttagccaggctggtctccaactcctgacttcagattatctgcccgccttggcctcccaaagtgctgggattacaggcgtgagcctccatacccggcccatgtcagatatatttaaaactaagaaagcttgggaaaatctctgccaatgatctccatatcagttaaccccgttccatagagtcagaaaggcagagggtcttagtgcagatgcctgcataaagataaaacgttgcatgttcttggaaaatatggctagaccacccttcccataccatctagctgcagtataaattaacatacccatgtggaaaagtggtatgaatcaagaactacaaaagtgttcatatacccttgactagaaattccacctccagtattttatcctaagaaaataatttatacacaaagacattcattgtggcattatgagatataatctaaactgttcaaaataagtaaaggttatatgaaacatggcacatccataacaatggagtaccataaaattaataatagttgacacagttttaatgacatggaataatgcctgtaggttgcggggaaaaaccccaagatataaattacactgagaatgatgaaactaagtaaaaatatgcagaagtagcaaagacaatggcaaggaagatgcaaaaatatcaagtgattttttctggtgacagaatcataggcaattaattgttatacttttctgtattgtctaaattttccacaataagcatgtactactgacataaacagaaaaaacaaacattattcaaccaggcaagcattaaagaatggacattgggtacagctttatttatttcttttaggaattgcaggttcctaacaaagtaggggtgaggggggtgttacaaaccagtcactaggcaggaacattagactccaaaagcagagaaatgcttaattttcttctacctgtttcaccacattcatgtagaactgtagtaaaaaagatggtgaatcaggctgaatcaatctaaataacaacttaaggctcccaaatcacatgaacctaggaccactaaatccaatgtcagacgtgtttaaatggtgcactgctctacatttttctattatgcaaagagctagaaaataatggtagtgtcattatgacattccatgaaaatgaagaaaatctttcaggaaaaattaagaaaataaaaatgtttactaaagaaagaatggtccggctaagtgcttttttttttttttttttttttaaaccaactgaaggccagagaaatgaaaggcatacccgtgaattaaattaatgctttaaaaaaaattgactttacttaaaatacaaacaaacgtcaactaatgaatactttattggcagaaaaaaaagacaacttggctggaaatgctgagtgtcttggactggtctgaaggaagaacatctgaaaggtctgaatgtcaaagtcagaacagtctctggtcaatcctactttgcttaaaatccaacattttacctttcttcaaattcctcaagactaaggaaaacttggttttataccaagaattatgaatcaacctacacttgctatcccttacatcacattttcattctagcttttctgaaacacattaccagataaatgccatataacctaaattcacctcaatgctttcattttgcctttacaattaccttaggacagatgccaagtttttataacttcaggccagaaaatcctcaagtggctcacctaattgtcagaaagtgagtgagtgacaacagacctcaggcacgaaactattttcagcaccaattacactgtggggggttaccagaacaagaaaaggccttcatagttctaagtgaagaaagataaaaacattttattttggccaggcgcggtggctcacgcctgtaaatcccagcactttgggaggccaaggcaggcggatcacctgaggtcgggagttcgagaccagcctgaccaaaatggagaaaccccgtatctactaaaaatacaaaattagctgggcgtggtgatacatgcctgtaatcccagctactcgggaggctgaggcaggagaatcgcttgaaccctgtaggtggaggttgcggtgagccaagatcgcaccattgcactccatcccgggcaacaagagcaagactcagcctcaaaaaaaaaaaaaaaaaaattgattttaggaggctgacaattacagttcatttcctaagatattccagacaatcactggttggctgacagaatctaggtgacagctaagatcacccctctgaaactcccttatatttggttaagcagaaatctgggctagcaaaataaactactagaaagtcagggtctggataagaaacagtgaccacattaaaggctgacggattaataatcatgatgttgccataaggccaaagtcataaagtactaatgctcaagacagataaacaacgtaagccccaatttcaagatgataaacttcaaagtgtattttttaaaatgcaagttgcctgtatgaaataaattaaaaatttatatgtaatttcagtgtaaaacaccaaaaccgaacattaaaactgttcacagaaaatagaaaaaaaaacaaaaaaacaaatcacaattataaaagcacagagatatcagttataagaaccaagtaaataaactaatttctattaatattttcatttactttataaaactttgttgattaaattgggggagtctctgacaatctaaagggtaacaaaataacaaatatacatcatttctttataagtcataccacacaaaccaagttaagttttttctatctgattacagagtcaataaatattgcatctgtatttagagcagcaacataaaactttattagaaagaaatactatatctggaccaaaaaactgcaacatggtttggaaatctaatgactaagaaggtaaaactggcaactatgtgcaactactgctcgtagatttgggtttgtttcccccccaacatctttaaaataagcagcccccacaaagggataatccattgaataaggagacaatgtagccaaagaagggatttgtggaaaaccatatgaatttaaatcaacataaaaagaacacacaaaggccatggaaacttgagaaggtgaaagaaaaaaaaaaaaaaccccaagcaaggacaagtcagctccttggagctgcaccaactcttaagtaggatgtccctattctaacggaaattgatgagtccacacctgggcacttcagtttgagaaatcaattggttggactggccattaaaaaaaggactttgtttttaaggtagataaagcttagagagagaaagctaaacagaaaagtaccaaatccttgtgaactcaaaaatgatttaggaagtcaaatgaagcaaactaaaaaactggatgaaaatgtttctctaagagtaaaacccagttttctctgtgatttaaaatcaaacaaacacactatagaagagaaattttcaaagtgcacccaataaaacctcagaggttccctggagtgtttggggtagcatggattgagacaggaagtgggttcaggcccatctcccccaacccttcttcactttaattcaaacatttctaattctcttttgtcgtttgtagtttcaggtaagatatcattttaaaaaaatgaaaaaaaaaaaaaatctaatgctgtccctttccctaagtttgaaaatcactgctgagactgaaattacattggtgagaaatatgatcatcataaatctaaaacacattttctatgtagtgctaccaaaatacaaagtttcatcaaatatttcactactattctgtaaaataaatgagaaaattaagttgttgggaagaaattaaattttgttattaccacctcccaaaatctgctcttctgctggctccaagatatcaatatttgatagtgtgaacaaatttctaacaaacattccagtcacaccgtaccccaaagacatttcattcaatggctgcatagtttcttttttgagaaggcaagcctcaaatttatagaaaactctagaatgaaaaatgtacaattactaaaaacataataacacactttatgtcagggcagaatctgcatagtgcttttaaacataatcaccaatgaagagtagccaaatcccagaacttcacacagcactcattagcaaacaacgtcaaagtgtaaatgataagcaggaaaaaaaccaagtaacacgaatgccatttttctttgatgcaatcacgaagaaaagtggaaatgcaggacgaaaagtggaatccaagctttggccacgtactgaaacttcattacttcaatgaaacagagcaaatctccatggaaaggactcattcagcaaacattaagttctttccatatattttttttccttcacgtaaggttaaacagaagttgctgtcattctagaatcagtgattacaattttttttttaattagaaaaaaggttacttgaatatttacataattttattgctctttattttaacaaaaacttttttcactgatttgtagactccatccattaacgtatgaaagtgaaatccatctctcaggaagatacagttatggttgaatgtatctgatgctgagagtacagcataattaagaaaaatccttgcatgtcatttggttcttgttgcagtcttctgtgttcacccctcagaaagcaaaagaatccatctgactttcaataaataccaaattattaaaaaaaaaaaaaaaagaacgtttccacagactagagatccaagaaaaagcagttctgatgaatgattcccagaatcaagtgagtcctcctttagtccaatgagatgatgtcaggaatgttacttccactgctggttatgacccctgtctcactcctgctgctggatgaactaacatgagtactgctttcatgggagctggtggtggtgacagacgtactgcttgctgttaagggtgaggtgagactatccaaaaacataggaggacagtactggggatcaactggaataagggaaagaaaatccaaacctgacaatatggcactagcaataataaggcagtcatatttttccttgaaataagctgttttccactccataaatacaaattatttgttttattttgtattcactgttgcacagtatcagaagatgttccaagcttcagttcattattaatatcatttcttctttgttctcctggcaaatctgatgacatgcttgatattggcgtatggtggaatggtactgagtagtctgttaatgaaggcggaatagcagcaggatcaaccgaagtcacactgggcacccttacagaagatggctgatacatgagaacccctttggttgggctgctttgtgtttctgacataaagatgcatttccttttggcaggagggtcttcctcttcgtcagaagagctttctattgtaagatcaataacatctactttcttcttgcttgcctcactggctacagtcactgaacaaggcttactgaggacgcttgaactttctatttttgtacacggttggctggatactttcatagcttctttcttcggtctcattggacaccaagaaccatcttcttggaatttgatctcatctacatcagaacagtcattgagaatttccataaaaagcccatctaatattagactttcataggcagcttttttgtcacacacaggacaaatccaggtgggctttttctcattcatttgtagatagagggcagcatcaaaacactgcagatgtgtacaagtcactgcacggcatgggattgtcagcctcatttttcctaaagggcacatcaaggatacccgaaggctagttgtagcaatttcactatcaggatctgcagtaagtttttctttaattagtgctctggaatgatcagggtttctaatacctttcatttttaatctctgtaataacatggctgatgtaagctgccgtacaagatatacagacatagagtaattcttcccaatttctgatgcccaagaaatggaaatttggtttggcacagctgaagataacctaactaaagatgtaatattcaaggggcgtccagggcgcttctgttcaatcccatttttaggcggtggtgcatagccaggcaaaggaaatagcttcccatttacttttatacatagactatttggatagttatcttcttgagggcaacttgtctctgccaggcaaagtctcaactgaacttggactgtataatctctcctaccacctggcaaaaaatccctggatatgcatatctctctaacttgttgaggtgtcaaagcaaaaataaaaaacttctcttgaaatcgctgaatactgctttgaactaaactcgtgggcttgatgagaacatcaaggacatcataaaagggcagattttttaactgcacatcaggatggacaggaggaattgggggagatggctgctgcatctcaaatgtgggcttagtatcttgaagcagcacagaaccaacaggagaggatggtgagtgaggtgtaactgaagtggaaggcaacgagtggattccagccacggccaagtcaggttctacaggtgatgagccaccatccaaactgaaaaccgatgatttgattgtggataaatcagaaagtccttcaagagttcgtggatatcggcgtctatacaattctcggattttaatctgaaccgcagggctgcagccgctcttcaataaatgcagcgccctcatcaggaggtcatgcttgcgtccacttttattccgtccagcaaagcctagtaatacttgtagttcagaaaccctaaaactagaaaccatattcctcaactcttcgaaatccgccattttataccacccgcgggcgccgccgccgctgccgccgcacccactcccgctgccgccaacgacgctgccgccaccacggccgccgccgcctccagcaccatcctgcactgggcgccgcttaagacgccgcggccgccgccgctacagccgggcccgtcacgt

SEQ ID NO: 13719 - RNA, 7755 nt, Homo sapiens
  source 1..7755: mol_type = other RNA
gctgggattacaggcatgagccaccatgcccagcttaagaattcttgatttttggaaccttgattataagctgcctgatgtctggaaccaaaacttctgtaacactctattccacgtgtacttacaaaacactctaaacatttattaaacagtttgatgaaggccaaaataagaggcatatgctattctacaacacggtaacactcttcgtcacttaaaataattaagctttgagaacacaaaataaagctttttaaaaaagccattcagaaataggaagcagtttgggaaatgattgtgctacgccaatcaagaaaatgttgtacctcaaacatctgaaggtagcaatctgtttttttctttccctgcagctacccttattggaaacataagggaatataaagtgaaaacaggcaatgtttgcctgtttttatagcttttagccttaccacttttcagtttggggatggaatgcctttggctcagtagattctactggctttggggagctcagaaaggccataatggggcctacaggaagaggaaaaagagagctgacctcttaagggcaggccttaggtacaagaggctttttttaaaaagtgacaaaacttttgaactaaagatggaaaacgtagtctgacaaagaatatttgtgcaactttacagtgccagtaaaatcatgggaaaagcttggatagccatacgtaggtgtttctgaaacatgtcagattttatatatatatatatatatatatatatatttttttttttttttttttttttttttagagagtcttgctttgttacccaggctggagtgcagtggcacaatctcggatcactgcaaatcctccgcctcctgggttcaagcgattctcctgcctcggtctcccaagtagctgggactacaggcgcctgccatcacacccacctaatttatgtttttgctagagatggggtttcaccatgttccatgttagccaggctggtctccaactcctgacttcagattatctgcccgccttggcctcccaaagtgctgggattacaggcgtgagcctccatacccggcccatgtcagatatatttaaaactaagaaagcttgggaaaatctctgccaatgatctccatatcagttaaccccgttccatagagtcagaaaggcagagggtcttagtgcagatgcctgcataaagataaaacgttgcatgttcttggaaaatatggctagaccacccttcccataccatctagctgcagtataaattaacatacccatgtggaaaagtggtatgaatcaagaactacaaaagtgttcatatacccttgactagaaattccacctccagtattttatcctaagaaaataatttatacacaaagacattcattgtggcattatgagatataatctaaactgttcaaaataagtaaaggttatatgaaacatggcacatccataacaatggagtaccataaaattaataatagttgacacagttttaatgacatggaataatgcctgtaggttgcggggaaaaaccccaagatataaattacactgagaatgatgaaactaagtaaaaatatgcagaagtagcaaagacaatggcaaggaagatgcaaaaatatcaagtgattttttctggtgacagaatcataggcaattaattgttatacttttctgtattgtctaaattttccacaataagcatgtactactgacataaacagaaaaaacaaacattattcaaccaggcaagcattaaagaatggacattgggtacagctttatttatttcttttaggaattgcaggttcctaacaaagtaggggtgaggggggtgttacaaaccagtcactaggcaggaacattagactccaaaagcagagaaatgcttaattttcttctacctgtttcaccacattcatgtagaactgtagtaaaaaagatggtgaatcaggctgaatcaatctaaataacaacttaaggctcccaaatcacatgaacctaggaccactaaatccaatgtcagacgtgtttaaatggtgcactgctctacatttttctattatgcaaagagctagaaaataatggtagtgtcattatgacattccatgaaaatgaagaaaatctttcaggaaaaattaagaaaataaaaatgtttactaaagaaagaatggtccggctaagtgcttttttttttttttttttttttaaaccaactgaaggccagagaaatgaaaggcatacccgtgaattaaattaatgctttaaaaaaaattgactttacttaaaatacaaacaaacgtcaactaatgaatactttattggcagaaaaaaaagacaacttggctggaaatgctgagtgtcttggactggtctgaaggaagaacatctgaaaggtctgaatgtcaaagtcagaacagtctctggtcaatcctactttgcttaaaatccaacattttacctttcttcaaattcctcaagactaaggaaaacttggttttataccaagaattatgaatcaacctacacttgctatcccttacatcacattttcattctagcttttctgaaacacattaccagataaatgccatataacctaaattcacctcaatgctttcattttgcctttacaattaccttaggacagatgccaagtttttataacttcaggccagaaaatcctcaagtggctcacctaattgtcagaaagtgagtgagtgacaacagacctcaggcacgaaactattttcagcaccaattacactgtggggggttaccagaacaagaaaaggccttcatagttctaagtgaagaaagataaaaacattttattttggccaggcgcggtggctcacgcctgtaaatcccagcactttgggaggccaaggcaggcggatcacctgaggtcgggagttcgagaccagcctgaccaaaatggagaaaccccgtatctactaaaaatacaaaattagctgggcgtggtgatacatgcctgtaatcccagctactcgggaggctgaggcaggagaatcgcttgaaccctgtaggtggaggttgcggtgagccaagatcgcaccattgcactccatcccgggcaacaagagcaagactcagcctcaaaaaaaaaaaaaaaaaaattgattttaggaggctgacaattacagttcatttcctaagatattccagacaatcactggttggctgacagaatctaggtgacagctaagatcacccctctgaaactcccttatatttggttaagcagaaatctgggctagcaaaataaactactagaaagtcagggtctggataagaaacagtgaccacattaaaggctgacggattaataatcatgatgttgccataaggccaaagtcataaagtactaatgctcaagacagataaacaacgtaagccccaatttcaagatgataaacttcaaagtgtattttttaaaatgcaagttgcctgtatgaaataaattaaaaatttatatgtaatttcagtgtaaaacaccaaaaccgaacattaaaactgttcacagaaaatagaaaaaaaaacaaaaaaacaaatcacaattataaaagcacagagatatcagttataagaaccaagtaaataaactaatttctattaatattttcatttactttataaaactttgttgattaaattgggggagtctctgacaatctaaagggtaacaaaataacaaatatacatcatttctttataagtcataccacacaaaccaagttaagttttttctatctgattacagagtcaataaatattgcatctgtatttagagcagcaacataaaactttattagaaagaaatactatatctggaccaaaaaactgcaacatggtttggaaatctaatgactaagaaggtaaaactggcaactatgtgcaactactgctcgtagatttgggtttgtttcccccccaacatctttaaaataagcagcccccacaaagggataatccattgaataaggagacaatgtagccaaagaagggatttgtggaaaaccatatgaatttaaatcaacataaaaagaacacacaaaggccatggaaacttgagaaggtgaaagaaaaaaaaaaaaaaccccaagcaaggacaagtcagctccttggagctgcaccaactcttaagtaggatgtccctattctaacggaaattgatgagtccacacctgggcacttcagtttgagaaatcaattggttggactggccattaaaaaaaggactttgtttttaaggtagataaagcttagagagagaaagctaaacagaaaagtaccaaatccttgtgaactcaaaaatgatttaggaagtcaaatgaagcaaactaaaaaactggatgaaaatgtttctctaagagtaaaacccagttttctctgtgatttaaaatcaaacaaacacactatagaagagaaattttcaaagtgcacccaataaaacctcagaggttccctggagtgtttggggtagcatggattgagacaggaagtgggttcaggcccatctcccccaacccttcttcactttaattcaaacatttctaattctcttttgtcgtttgtagtttcaggtaagatatcattttaaaaaaatgaaaaaaaaaaaaaatctaatgctgtccctttccctaagtttgaaaatcactgctgagactgaaattacattggtgagaaatatgatcatcataaatctaaaacacattttctatgtagtgctaccaaaatacaaagtttcatcaaatatttcactactattctgtaaaataaatgagaaaattaagttgttgggaagaaattaaattttgttattaccacctcccaaaatctgctcttctgctggctccaagatatcaatatttgatagtgtgaacaaatttctaacaaacattccagtcacaccgtaccccaaagacatttcattcaatggctgcatagtttcttttttgagaaggcaagcctcaaatttatagaaaactctagaatgaaaaatgtacaattactaaaaacataataacacactttatgtcagggcagaatctgcatagtgcttttaaacataatcaccaatgaagagtagccaaatcccagaacttcacacagcactcattagcaaacaacgtcaaagtgtaaatgataagcaggaaaaaaaccaagtaacacgaatgccatttttctttgatgcaatcacgaagaaaagtggaaatgcaggacgaaaagtggaatccaagctttggccacgtactgaaacttcattacttcaatgaaacagagcaaatctccatggaaaggactcattcagcaaacattaagttctttccatatattttttttccttcacgtaaggttaaacagaagttgctgtcattctagaatcagtgattacaattttttttttaattagaaaaaaggttacttgaatatttacataattttattgctctttattttaacaaaaacttttttcactgatttgtagactccatccattaacgtatgaaagtgaaatccatctctcaggaagatacagttatggttgaatgtatctgatgctgagagtacagcataattaagaaaaatccttgcatgtcatttggttcttgttgcagtcttctgtgttcacccctcagaaagcaaaagaatccatctgactttcaataaataccaaattattaaaaaaaaaaaaaaaagaacgtttccacagactagagatccaagaaaaagcagttctgatgaatgattcccagaatcaagtgagtcctcctttagtccaatgagatgatgtcaggaatgttacttccactgctggttatgacccctgtctcactcctgctgctggatgaactaacatgagtactgctttcatgggagctggtggtggtgacagacgtactgcttgctgttaagggtgaggtgagactatccaaaaacataggaggacagtactggggatcaactggaataagggaaagaaaatccaaacctggcaaatctgatgacatgcttgatattggcgtatggtggaatggtactgagtagtctgttaatgaaggcggaatagcagcaggatcaaccgaagtcacactgggcacccttacagaagatggctgatacatgagaacccctttggttgggctgctttgtgtttctgacataaagatgcatttccttttggcaggagggtcttcctcttcgtcagaagagctttctattgtaagatcaataacatctactttcttcttgcttgcctcactggctacagtcactgaacaaggcttactgaggacgcttgaactttctatttttgtacacggttggctggatactttcatagcttctttcttcggtctcattggacaccaagaaccatcttcttggaatttgatctcatctacatcagaacagtcattgagaatttccataaaaagcccatctaatattagactttcataggcagcttttttgtcacacacaggacaaatccaggtgggctttttctcattcatttgtagatagagggcagcatcaaaacactgcagatgtgtacaagtcactgcacggcatgggattgtcagcctcatttttcctaaagggcacatcaaggatacccgaaggctagttgtagcaatttcactatcaggatctgcagtaagtttttctttaattagtgctctggaatgatcagggtttctaatacctttcatttttaatctctgtaataacatggctgatgtaagctgccgtacaagatatacagacatagagtaattcttcccaatttctgatgcccaagaaatggaaatttggtttggcacagctgaagataacctaactaaagatgtaatattcaaggggcgtccagggcgcttctgttcaatcccatttttaggcggtggtgcatagccaggcaaaggaaatagcttcccatttacttttatacatagactatttggatagttatcttcttgagggcaacttgtctctgccaggcaaagtctcaactgaacttggactgtataatctctcctaccacctggcaaaaaatccctaaactcgtgggcttgatgagaacatcaaggacatcataaaagggcagattttttaactgcacatcaggatggacaggaggaattgggggagatggctgctgcatctcaaatgtgggcttagtatcttgaagcagcacagaaccaacaggagaggatggtgagtgaggtgtaactgaagtggaaggcaacgagtggattccagccacggccaagtcaggttctacaggtgatgagccaccatccaaactgaaaaccgatgatttgattgtggataaatcagaaagtccttcaagagttcgtggatatcggcgtctatacaattctcggattttaatctgaaccgcagggctgcagccgctcttcaataaatgcagcgccctcatcaggaggtcatgcttgcgtccacttttattccgtccagcaaagcctagtaatacttgtagttcagaaaccctaaaactagaaaccatattcctcaactcttcgaaatccgccattttataccacccgcgggcgccgccgccgctgccgccgcacccactcccgctgccgccaacgacgctgccgccaccacggccgccgccgcctccagcaccatcctgcactgggcgccgcttaagacgccgcggccgccgccgctacagccgggcccgtcacgt

SEQ ID NO: 13720 - RNA, 7949 nt, Homo sapiens
  source 1..7949: mol_type = other RNA
gctgggattacaggcatgagccaccatgcccagcttaagaattcttgatttttggaaccttgattataagctgcctgatgtctggaaccaaaacttctgtaacactctattccacgtgtacttacaaaacactctaaacatttattaaacagtttgatgaaggccaaaataagaggcatatgctattctacaacacggtaacactcttcgtcacttaaaataattaagctttgagaacacaaaataaagctttttaaaaaagccattcagaaataggaagcagtttgggaaatgattgtgctacgccaatcaagaaaatgttgtacctcaaacatctgaaggtagcaatctgtttttttctttccctgcagctacccttattggaaacataagggaatataaagtgaaaacaggcaatgtttgcctgtttttatagcttttagccttaccacttttcagtttggggatggaatgcctttggctcagtagattctactggctttggggagctcagaaaggccataatggggcctacaggaagaggaaaaagagagctgacctcttaagggcaggccttaggtacaagaggctttttttaaaaagtgacaaaacttttgaactaaagatggaaaacgtagtctgacaaagaatatttgtgcaactttacagtgccagtaaaatcatgggaaaagcttggatagccatacgtaggtgtttctgaaacatgtcagattttatatatatatatatatatatatatatatttttttttttttttttttttttttttagagagtcttgctttgttacccaggctggagtgcagtggcacaatctcggatcactgcaaatcctccgcctcctgggttcaagcgattctcctgcctcggtctcccaagtagctgggactacaggcgcctgccatcacacccacctaatttatgtttttgctagagatggggtttcaccatgttccatgttagccaggctggtctccaactcctgacttcagattatctgcccgccttggcctcccaaagtgctgggattacaggcgtgagcctccatacccggcccatgtcagatatatttaaaactaagaaagcttgggaaaatctctgccaatgatctccatatcagttaaccccgttccatagagtcagaaaggcagagggtcttagtgcagatgcctgcataaagataaaacgttgcatgttcttggaaaatatggctagaccacccttcccataccatctagctgcagtataaattaacatacccatgtggaaaagtggtatgaatcaagaactacaaaagtgttcatatacccttgactagaaattccacctccagtattttatcctaagaaaataatttatacacaaagacattcattgtggcattatgagatataatctaaactgttcaaaataagtaaaggttatatgaaacatggcacatccataacaatggagtaccataaaattaataatagttgacacagttttaatgacatggaataatgcctgtaggttgcggggaaaaaccccaagatataaattacactgagaatgatgaaactaagtaaaaatatgcagaagtagcaaagacaatggcaaggaagatgcaaaaatatcaagtgattttttctggtgacagaatcataggcaattaattgttatacttttctgtattgtctaaattttccacaataagcatgtactactgacataaacagaaaaaacaaacattattcaaccaggcaagcattaaagaatggacattgggtacagctttatttatttcttttaggaattgcaggttcctaacaaagtaggggtgaggggggtgttacaaaccagtcactaggcaggaacattagactccaaaagcagagaaatgcttaattttcttctacctgtttcaccacattcatgtagaactgtagtaaaaaagatggtgaatcaggctgaatcaatctaaataacaacttaaggctcccaaatcacatgaacctaggaccactaaatccaatgtcagacgtgtttaaatggtgcactgctctacatttttctattatgcaaagagctagaaaataatggtagtgtcattatgacattccatgaaaatgaagaaaatctttcaggaaaaattaagaaaataaaaatgtttactaaagaaagaatggtccggctaagtgcttttttttttttttttttttttaaaccaactgaaggccagagaaatgaaaggcatacccgtgaattaaattaatgctttaaaaaaaattgactttacttaaaatacaaacaaacgtcaactaatgaatactttattggcagaaaaaaaagacaacttggctggaaatgctgagtgtcttggactggtctgaaggaagaacatctgaaaggtctgaatgtcaaagtcagaacagtctctggtcaatcctactttgcttaaaatccaacattttacctttcttcaaattcctcaagactaaggaaaacttggttttataccaagaattatgaatcaacctacacttgctatcccttacatcacattttcattctagcttttctgaaacacattaccagataaatgccatataacctaaattcacctcaatgctttcattttgcctttacaattaccttaggacagatgccaagtttttataacttcaggccagaaaatcctcaagtggctcacctaattgtcagaaagtgagtgagtgacaacagacctcaggcacgaaactattttcagcaccaattacactgtggggggttaccagaacaagaaaaggccttcatagttctaagtgaagaaagataaaaacattttattttggccaggcgcggtggctcacgcctgtaaatcccagcactttgggaggccaaggcaggcggatcacctgaggtcgggagttcgagaccagcctgaccaaaatggagaaaccccgtatctactaaaaatacaaaattagctgggcgtggtgatacatgcctgtaatcccagctactcgggaggctgaggcaggagaatcgcttgaaccctgtaggtggaggttgcggtgagccaagatcgcaccattgcactccatcccgggcaacaagagcaagactcagcctcaaaaaaaaaaaaaaaaaaattgattttaggaggctgacaattacagttcatttcctaagatattccagacaatcactggttggctgacagaatctaggtgacagctaagatcacccctctgaaactcccttatatttggttaagcagaaatctgggctagcaaaataaactactagaaagtcagggtctggataagaaacagtgaccacattaaaggctgacggattaataatcatgatgttgccataaggccaaagtcataaagtactaatgctcaagacagataaacaacgtaagccccaatttcaagatgataaacttcaaagtgtattttttaaaatgcaagttgcctgtatgaaataaattaaaaatttatatgtaatttcagtgtaaaacaccaaaaccgaacattaaaactgttcacagaaaatagaaaaaaaaacaaaaaaacaaatcacaattataaaagcacagagatatcagttataagaaccaagtaaataaactaatttctattaatattttcatttactttataaaactttgttgattaaattgggggagtctctgacaatctaaagggtaacaaaataacaaatatacatcatttctttataagtcataccacacaaaccaagttaagttttttctatctgattacagagtcaataaatattgcatctgtatttagagcagcaacataaaactttattagaaagaaatactatatctggaccaaaaaactgcaacatggtttggaaatctaatgactaagaaggtaaaactggcaactatgtgcaactactgctcgtagatttgggtttgtttcccccccaacatctttaaaataagcagcccccacaaagggataatccattgaataaggagacaatgtagccaaagaagggatttgtggaaaaccatatgaatttaaatcaacataaaaagaacacacaaaggccatggaaacttgagaaggtgaaagaaaaaaaaaaaaaaccccaagcaaggacaagtcagctccttggagctgcaccaactcttaagtaggatgtccctattctaacggaaattgatgagtccacacctgggcacttcagtttgagaaatcaattggttggactggccattaaaaaaaggactttgtttttaaggtagataaagcttagagagagaaagctaaacagaaaagtaccaaatccttgtgaactcaaaaatgatttaggaagtcaaatgaagcaaactaaaaaactggatgaaaatgtttctctaagagtaaaacccagttttctctgtgatttaaaatcaaacaaacacactatagaagagaaattttcaaagtgcacccaataaaacctcagaggttccctggagtgtttggggtagcatggattgagacaggaagtgggttcaggcccatctcccccaacccttcttcactttaattcaaacatttctaattctcttttgtcgtttgtagtttcaggtaagatatcattttaaaaaaatgaaaaaaaaaaaaaatctaatgctgtccctttccctaagtttgaaaatcactgctgagactgaaattacattggtgagaaatatgatcatcataaatctaaaacacattttctatgtagtgctaccaaaatacaaagtttcatcaaatatttcactactattctgtaaaataaatgagaaaattaagttgttgggaagaaattaaattttgttattaccacctcccaaaatctgctcttctgctggctccaagatatcaatatttgatagtgtgaacaaatttctaacaaacattccagtcacaccgtaccccaaagacatttcattcaatggctgcatagtttcttttttgagaaggcaagcctcaaatttatagaaaactctagaatgaaaaatgtacaattactaaaaacataataacacactttatgtcagggcagaatctgcatagtgcttttaaacataatcaccaatgaagagtagccaaatcccagaacttcacacagcactcattagcaaacaacgtcaaagtgtaaatgataagcaggaaaaaaaccaagtaacacgaatgccatttttctttgatgcaatcacgaagaaaagtggaaatgcaggacgaaaagtggaatccaagctttggccacgtactgaaacttcattacttcaatgaaacagagcaaatctccatggaaaggactcattcagcaaacattaagttctttccatatattttttttccttcacgtaaggttaaacagaagttgctgtcattctagaatcagtgattacaattttttttttaattagaaaaaaggttacttgaatatttacataattttattgctctttattttaacaaaaacttttttcactgatttgtagactccatccattaacgtatgaaagtgaaatccatctctcaggaagatacagttatggttgaatgtatctgatgctgagagtacagcataattaagaaaaatccttgcatgtcatttggttcttgttgcagtcttctgtgttcacccctcagaaagcaaaagaatccatctgactttcaataaataccaaattattaaaaaaaaaaaaaaaagaacgtttccacagactagagatccaagaaaaagcagttctgatgaatgattcccagaatcaagtgagtcctcctttagtccaatgagatgatgtcaggaatgttacttccactgctggttatgacccctgtctcactcctgctgctggatgaactaacatgagtactgctttcatgggagctggtggtggtgacagacgtactgcttgctgttaagggtgaggtgagactatccaaaaacataggaggacagtactggggatcaactggaataagggaaagaaaatccaaacctggcaaatctgatgacatgcttgatattggcgtatggtggaatggtactgagtagtctgttaatgaaggcggaatagcagcaggatcaaccgaagtcacactgggcacccttacagaagatggctgatacatgagaacccctttggttgggctgctttgtgtttctgacataaagatgcatttccttttggcaggagggtcttcctcttcgtcagaagagctttctattgtaagatcaataacatctactttcttcttgcttgcctcactggctacagtcactgaacaaggcttactgaggacgcttgaactttctatttttgtacacggttggctggatactttcatagcttctttcttcggtctcattggacaccaagaaccatcttcttggaatttgatctcatctacatcagaacagtcattgagaatttccataaaaagcccatctaatattagactttcataggcagcttttttgtcacacacaggacaaatccaggtgggctttttctcattcatttgtagatagagggcagcatcaaaacactgcagatgtgtacaagtcactgcacggcatgggattgtcagcctcatttttcctaaagggcacatcaaggatacccgaaggctagttgtagcaatttcactatcaggatctgcagtaagtttttctttaattagtgctctggaatgatcagggtttctaatacctttcatttttaatctctgtaataacatggctgatgtaagctgccgtacaagatatacagacatagagtaattcttcccaatttctgatgcccaagaaatggaaatttggtttggcacagctgaagataacctaactaaagatgtaatattcaaggggcgtccagggcgcttctgttcaatcccatttttaggcggtggtgcatagccaggcaaaggaaatagcttcccatttacttttatacatagactatttggatagttatcttcttgagggcaacttgtctctgccaggcaaagtctcaactgaacttggactgtataatctctcctaccacctggcaaaaaatccctggatatgcatatctctctaacttgttgaggtgtcaaagcaaaaataaaaaacttctcttgaaatcgctgaatactgctttgaactaaactcgtgggcttgatgagaacatcaaggacatcataaaagggcagattttttaactgcacatcaggatggacaggaggaattgggggagatggctgctgcatctcaaatgtgggcttagtatcttgaagcagcacagaaccaacaggagaggatggtgagtgaggtgtaactgaagtggaaggcaacgagtggattccagccacggccaagtcaggttctacaggtgatgagccaccatccaaactgaaaaccgatgatttgattgtggataaatcagaaagtccttcaagagttcgtggatatcggcgtctatacaattctcggattttaatctgaaccgcagggctgcagccgctcttcaataaatgcagcgccctcatcaggaggtcatgcttgcgtccacttttattccgtccagcaaagcctagtaatacttgtagttcagaaaccctaaaactagaaaccatattcagaatggctaaaatgaaaaacactgataacaccaaatgctggcgaggatgctgagaaactggatcactccatacattgctggtagggatgtaaaatggtacagccactcctcaactcttcgaaatccgccattttataccacccgcgggcgccgccgccgctgccgccgcacccactcccgctgccgccaacgacgctgccgccaccacggccgccgccgcctccagcaccatcctgcactgggcgccgcttaagacgccgcggccgccgccgctacagccgggcccgtcacgt

SEQ ID NO: 13721 - RNA, 8038 nt, Homo sapiens
  source 1..8038: mol_type = other RNA
gctgggattacaggcatgagccaccatgcccagcttaagaattcttgatttttggaaccttgattataagctgcctgatgtctggaaccaaaacttctgtaacactctattccacgtgtacttacaaaacactctaaacatttattaaacagtttgatgaaggccaaaataagaggcatatgctattctacaacacggtaacactcttcgtcacttaaaataattaagctttgagaacacaaaataaagctttttaaaaaagccattcagaaataggaagcagtttgggaaatgattgtgctacgccaatcaagaaaatgttgtacctcaaacatctgaaggtagcaatctgtttttttctttccctgcagctacccttattggaaacataagggaatataaagtgaaaacaggcaatgtttgcctgtttttatagcttttagccttaccacttttcagtttggggatggaatgcctttggctcagtagattctactggctttggggagctcagaaaggccataatggggcctacaggaagaggaaaaagagagctgacctcttaagggcaggccttaggtacaagaggctttttttaaaaagtgacaaaacttttgaactaaagatggaaaacgtagtctgacaaagaatatttgtgcaactttacagtgccagtaaaatcatgggaaaagcttggatagccatacgtaggtgtttctgaaacatgtcagattttatatatatatatatatatatatatatatttttttttttttttttttttttttttagagagtcttgctttgttacccaggctggagtgcagtggcacaatctcggatcactgcaaatcctccgcctcctgggttcaagcgattctcctgcctcggtctcccaagtagctgggactacaggcgcctgccatcacacccacctaatttatgtttttgctagagatggggtttcaccatgttccatgttagccaggctggtctccaactcctgacttcagattatctgcccgccttggcctcccaaagtgctgggattacaggcgtgagcctccatacccggcccatgtcagatatatttaaaactaagaaagcttgggaaaatctctgccaatgatctccatatcagttaaccccgttccatagagtcagaaaggcagagggtcttagtgcagatgcctgcataaagataaaacgttgcatgttcttggaaaatatggctagaccacccttcccataccatctagctgcagtataaattaacatacccatgtggaaaagtggtatgaatcaagaactacaaaagtgttcatatacccttgactagaaattccacctccagtattttatcctaagaaaataatttatacacaaagacattcattgtggcattatgagatataatctaaactgttcaaaataagtaaaggttatatgaaacatggcacatccataacaatggagtaccataaaattaataatagttgacacagttttaatgacatggaataatgcctgtaggttgcggggaaaaaccccaagatataaattacactgagaatgatgaaactaagtaaaaatatgcagaagtagcaaagacaatggcaaggaagatgcaaaaatatcaagtgattttttctggtgacagaatcataggcaattaattgttatacttttctgtattgtctaaattttccacaataagcatgtactactgacataaacagaaaaaacaaacattattcaaccaggcaagcattaaagaatggacattgggtacagctttatttatttcttttaggaattgcaggttcctaacaaagtaggggtgaggggggtgttacaaaccagtcactaggcaggaacattagactccaaaagcagagaaatgcttaattttcttctacctgtttcaccacattcatgtagaactgtagtaaaaaagatggtgaatcaggctgaatcaatctaaataacaacttaaggctcccaaatcacatgaacctaggaccactaaatccaatgtcagacgtgtttaaatggtgcactgctctacatttttctattatgcaaagagctagaaaataatggtagtgtcattatgacattccatgaaaatgaagaaaatctttcaggaaaaattaagaaaataaaaatgtttactaaagaaagaatggtccggctaagtgcttttttttttttttttttttttaaaccaactgaaggccagagaaatgaaaggcatacccgtgaattaaattaatgctttaaaaaaaattgactttacttaaaatacaaacaaacgtcaactaatgaatactttattggcagaaaaaaaagacaacttggctggaaatgctgagtgtcttggactggtctgaaggaagaacatctgaaaggtctgaatgtcaaagtcagaacagtctctggtcaatcctactttgcttaaaatccaacattttacctttcttcaaattcctcaagactaaggaaaacttggttttataccaagaattatgaatcaacctacacttgctatcccttacatcacattttcattctagcttttctgaaacacattaccagataaatgccatataacctaaattcacctcaatgctttcattttgcctttacaattaccttaggacagatgccaagtttttataacttcaggccagaaaatcctcaagtggctcacctaattgtcagaaagtgagtgagtgacaacagacctcaggcacgaaactattttcagcaccaattacactgtggggggttaccagaacaagaaaaggccttcatagttctaagtgaagaaagataaaaacattttattttggccaggcgcggtggctcacgcctgtaaatcccagcactttgggaggccaaggcaggcggatcacctgaggtcgggagttcgagaccagcctgaccaaaatggagaaaccccgtatctactaaaaatacaaaattagctgggcgtggtgatacatgcctgtaatcccagctactcgggaggctgaggcaggagaatcgcttgaaccctgtaggtggaggttgcggtgagccaagatcgcaccattgcactccatcccgggcaacaagagcaagactcagcctcaaaaaaaaaaaaaaaaaaattgattttaggaggctgacaattacagttcatttcctaagatattccagacaatcactggttggctgacagaatctaggtgacagctaagatcacccctctgaaactcccttatatttggttaagcagaaatctgggctagcaaaataaactactagaaagtcagggtctggataagaaacagtgaccacattaaaggctgacggattaataatcatgatgttgccataaggccaaagtcataaagtactaatgctcaagacagataaacaacgtaagccccaatttcaagatgataaacttcaaagtgtattttttaaaatgcaagttgcctgtatgaaataaattaaaaatttatatgtaatttcagtgtaaaacaccaaaaccgaacattaaaactgttcacagaaaatagaaaaaaaaacaaaaaaacaaatcacaattataaaagcacagagatatcagttataagaaccaagtaaataaactaatttctattaatattttcatttactttataaaactttgttgattaaattgggggagtctctgacaatctaaagggtaacaaaataacaaatatacatcatttctttataagtcataccacacaaaccaagttaagttttttctatctgattacagagtcaataaatattgcatctgtatttagagcagcaacataaaactttattagaaagaaatactatatctggaccaaaaaactgcaacatggtttggaaatctaatgactaagaaggtaaaactggcaactatgtgcaactactgctcgtagatttgggtttgtttcccccccaacatctttaaaataagcagcccccacaaagggataatccattgaataaggagacaatgtagccaaagaagggatttgtggaaaaccatatgaatttaaatcaacataaaaagaacacacaaaggccatggaaacttgagaaggtgaaagaaaaaaaaaaaaaaccccaagcaaggacaagtcagctccttggagctgcaccaactcttaagtaggatgtccctattctaacggaaattgatgagtccacacctgggcacttcagtttgagaaatcaattggttggactggccattaaaaaaaggactttgtttttaaggtagataaagcttagagagagaaagctaaacagaaaagtaccaaatccttgtgaactcaaaaatgatttaggaagtcaaatgaagcaaactaaaaaactggatgaaaatgtttctctaagagtaaaacccagttttctctgtgatttaaaatcaaacaaacacactatagaagagaaattttcaaagtgcacccaataaaacctcagaggttccctggagtgtttggggtagcatggattgagacaggaagtgggttcaggcccatctcccccaacccttcttcactttaattcaaacatttctaattctcttttgtcgtttgtagtttcaggtaagatatcattttaaaaaaatgaaaaaaaaaaaaaatctaatgctgtccctttccctaagtttgaaaatcactgctgagactgaaattacattggtgagaaatatgatcatcataaatctaaaacacattttctatgtagtgctaccaaaatacaaagtttcatcaaatatttcactactattctgtaaaataaatgagaaaattaagttgttgggaagaaattaaattttgttattaccacctcccaaaatctgctcttctgctggctccaagatatcaatatttgatagtgtgaacaaatttctaacaaacattccagtcacaccgtaccccaaagacatttcattcaatggctgcatagtttcttttttgagaaggcaagcctcaaatttatagaaaactctagaatgaaaaatgtacaattactaaaaacataataacacactttatgtcagggcagaatctgcatagtgcttttaaacataatcaccaatgaagagtagccaaatcccagaacttcacacagcactcattagcaaacaacgtcaaagtgtaaatgataagcaggaaaaaaaccaagtaacacgaatgccatttttctttgatgcaatcacgaagaaaagtggaaatgcaggacgaaaagtggaatccaagctttggccacgtactgaaacttcattacttcaatgaaacagagcaaatctccatggaaaggactcattcagcaaacattaagttctttccatatattttttttccttcacgtaaggttaaacagaagttgctgtcattctagaatcagtgattacaattttttttttaattagaaaaaaggttacttgaatatttacataattttattgctctttattttaacaaaaacttttttcactgatttgtagactccatccattaacgtatgaaagtgaaatccatctctcaggaagatacagttatggttgaatgtatctgatgctgagagtacagcataattaagaaaaatccttgcatgtcatttggttcttgttgcagtcttctgtgttcacccctcagaaagcaaaagaatccatctgactttcaataaataccaaattattaaaaaaaaaaaaaaaagaacgtttccacagactagagatccaagaaaaagcagttctgatgaatgattcccagaatcaagtgagtcctcctttagtccaatgagatgatgtcaggaatgttacttccactgctggttatgacccctgtctcactcctgctgctggatgaactaacatgagtactgctttcatgggagctggtggtggtgacagacgtactgcttgctgttaagggtgaggtgagactatccaaaaacataggaggacagtactggggatcaactggaataagggaaagaaaatccaaacctggcaaatctgatgacatgcttgatattggcgtatggtggaatggtactgagtagtctgttaatgaaggcggaatagcagcaggatcaaccgaagtcacactgggcacccttacagaagatggctgatacatgagaacccctttggttgggctgctttgtgtttctgacataaagatgcatttccttttggcaggagggtcttcctcttcgtcagaagagctttctattgtaagatcaataacatctactttcttcttgcttgcctcactggctacagtcactgaacaaggcttactgaggacgcttgaactttctatttttgtacacggttggctggatactttcatagcttctttcttcggtctcattggacaccaagaaccatcttcttggaatttgatctcatctacatcagaacagtcattgagaatttccataaaaagcccatctaatattagactttcataggcagcttttttgtcacacacaggacaaatccaggtgggctttttctcattcatttgtagatagagggcagcatcaaaacactgcagatgtgtacaagtcactgcacggcatgggattgtcagcctcatttttcctaaagggcacatcaaggatacccgaaggctagttgtagcaatttcactatcaggatctgcagtaagtttttctttaattagtgctctggaatgatcagggtttctaatacctttcatttttaatctctgtaataacatggctgatgtaagctgccgtacaagatatacagacatagagtaattcttcccaatttctgatgcccaagaaatggaaatttggtttggcacagctgaagataacctaactaaagatgtaatattcaaggggcgtccagggcgcttctgttcaatcccatttttaggcggtggtgcatagccaggcaaaggaaatagcttcccatttacttttatacatagactatttggatagttatcttcttgagggcaacttgtctctgccaggcaaagtctcaactgaacttggactgtataatctctcctaccacctggcaaaaaatccctggatatgcatatctctctaacttgttgaggtgtcaaagcaaaaataaaaaacttctcttgaaatcgctgaatactgctttgaactaaactcgtgggcttgatgagaacatcaaggacatcataaaagggcagattttttaactgcacatcaggatggacaggaggaattgggggagatggctgctgcatctcaaatgtgggcttagtatcttgaagcagcacagaaccaacaggagaggatggtgagtgaggtgtaactgaagtggaaggcaacgagtggattccagccacggccaagtcaggttctacaggtgatgagccaccatccaaactgaaaaccgatgatttgattgtggataaatcagaaagtccttcaagagttcgtggatatcggcgtctatacaattctcggattttaatctgaaccgcagggctgcagccgctcttcaataaatgcagcgccctcatcaggaggtcatgcttgcgtccacttttattccgtccagcaaagcctagtaatacttgtagttcagaaaccctaaaactagaaaccatattcagaatggctaaaatgaaaaacactgataacaccaaatgctggcgaggatgctgagaaactggatcactccatacattgctggtagggatgtaaaatggtacagccacttgtgaaactttgaaagcattccctttaaaatcaggaacaagatcaggatgcccccatcacagcttctattcaacattgtactggagatccctcaactcttcgaaatccgccattttataccacccgcgggcgccgccgccgctgccgccgcacccactcccgctgccgccaacgacgctgccgccaccacggccgccgccgcctccagcaccatcctgcactgggcgccgcttaagacgccgcggccgccgccgctacagccgggcccgtcacgt

SEQ ID NO: 13722 - RNA, 7840 nt, Homo sapiens
  source 1..7840: mol_type = other RNA
gctgggattacaggcatgagccaccatgcccagcttaagaattcttgatttttggaaccttgattataagctgcctgatgtctggaaccaaaacttctgtaacactctattccacgtgtacttacaaaacactctaaacatttattaaacagtttgatgaaggccaaaataagaggcatatgctattctacaacacggtaacactcttcgtcacttaaaataattaagctttgagaacacaaaataaagctttttaaaaaagccattcagaaataggaagcagtttgggaaatgattgtgctacgccaatcaagaaaatgttgtacctcaaacatctgaaggtagcaatctgtttttttctttccctgcagctacccttattggaaacataagggaatataaagtgaaaacaggcaatgtttgcctgtttttatagcttttagccttaccacttttcagtttggggatggaatgcctttggctcagtagattctactggctttggggagctcagaaaggccataatggggcctacaggaagaggaaaaagagagctgacctcttaagggcaggccttaggtacaagaggctttttttaaaaagtgacaaaacttttgaactaaagatggaaaacgtagtctgacaaagaatatttgtgcaactttacagtgccagtaaaatcatgggaaaagcttggatagccatacgtaggtgtttctgaaacatgtcagattttatatatatatatatatatatatatatatttttttttttttttttttttttttttagagagtcttgctttgttacccaggctggagtgcagtggcacaatctcggatcactgcaaatcctccgcctcctgggttcaagcgattctcctgcctcggtctcccaagtagctgggactacaggcgcctgccatcacacccacctaatttatgtttttgctagagatggggtttcaccatgttccatgttagccaggctggtctccaactcctgacttcagattatctgcccgccttggcctcccaaagtgctgggattacaggcgtgagcctccatacccggcccatgtcagatatatttaaaactaagaaagcttgggaaaatctctgccaatgatctccatatcagttaaccccgttccatagagtcagaaaggcagagggtcttagtgcagatgcctgcataaagataaaacgttgcatgttcttggaaaatatggctagaccacccttcccataccatctagctgcagtataaattaacatacccatgtggaaaagtggtatgaatcaagaactacaaaagtgttcatatacccttgactagaaattccacctccagtattttatcctaagaaaataatttatacacaaagacattcattgtggcattatgagatataatctaaactgttcaaaataagtaaaggttatatgaaacatggcacatccataacaatggagtaccataaaattaataatagttgacacagttttaatgacatggaataatgcctgtaggttgcggggaaaaaccccaagatataaattacactgagaatgatgaaactaagtaaaaatatgcagaagtagcaaagacaatggcaaggaagatgcaaaaatatcaagtgattttttctggtgacagaatcataggcaattaattgttatacttttctgtattgtctaaattttccacaataagcatgtactactgacataaacagaaaaaacaaacattattcaaccaggcaagcattaaagaatggacattgggtacagctttatttatttcttttaggaattgcaggttcctaacaaagtaggggtgaggggggtgttacaaaccagtcactaggcaggaacattagactccaaaagcagagaaatgcttaattttcttctacctgtttcaccacattcatgtagaactgtagtaaaaaagatggtgaatcaggctgaatcaatctaaataacaacttaaggctcccaaatcacatgaacctaggaccactaaatccaatgtcagacgtgtttaaatggtgcactgctctacatttttctattatgcaaagagctagaaaataatggtagtgtcattatgacattccatgaaaatgaagaaaatctttcaggaaaaattaagaaaataaaaatgtttactaaagaaagaatggtccggctaagtgcttttttttttttttttttttttaaaccaactgaaggccagagaaatgaaaggcatacccgtgaattaaattaatgctttaaaaaaaattgactttacttaaaatacaaacaaacgtcaactaatgaatactttattggcagaaaaaaaagacaacttggctggaaatgctgagtgtcttggactggtctgaaggaagaacatctgaaaggtctgaatgtcaaagtcagaacagtctctggtcaatcctactttgcttaaaatccaacattttacctttcttcaaattcctcaagactaaggaaaacttggttttataccaagaattatgaatcaacctacacttgctatcccttacatcacattttcattctagcttttctgaaacacattaccagataaatgccatataacctaaattcacctcaatgctttcattttgcctttacaattaccttaggacagatgccaagtttttataacttcaggccagaaaatcctcaagtggctcacctaattgtcagaaagtgagtgagtgacaacagacctcaggcacgaaactattttcagcaccaattacactgtggggggttaccagaacaagaaaaggccttcatagttctaagtgaagaaagataaaaacattttattttggccaggcgcggtggctcacgcctgtaaatcccagcactttgggaggccaaggcaggcggatcacctgaggtcgggagttcgagaccagcctgaccaaaatggagaaaccccgtatctactaaaaatacaaaattagctgggcgtggtgatacatgcctgtaatcccagctactcgggaggctgaggcaggagaatcgcttgaaccctgtaggtggaggttgcggtgagccaagatcgcaccattgcactccatcccgggcaacaagagcaagactcagcctcaaaaaaaaaaaaaaaaaaattgattttaggaggctgacaattacagttcatttcctaagatattccagacaatcactggttggctgacagaatctaggtgacagctaagatcacccctctgaaactcccttatatttggttaagcagaaatctgggctagcaaaataaactactagaaagtcagggtctggataagaaacagtgaccacattaaaggctgacggattaataatcatgatgttgccataaggccaaagtcataaagtactaatgctcaagacagataaacaacgtaagccccaatttcaagatgataaacttcaaagtgtattttttaaaatgcaagttgcctgtatgaaataaattaaaaatttatatgtaatttcagtgtaaaacaccaaaaccgaacattaaaactgttcacagaaaatagaaaaaaaaacaaaaaaacaaatcacaattataaaagcacagagatatcagttataagaaccaagtaaataaactaatttctattaatattttcatttactttataaaactttgttgattaaattgggggagtctctgacaatctaaagggtaacaaaataacaaatatacatcatttctttataagtcataccacacaaaccaagttaagttttttctatctgattacagagtcaataaatattgcatctgtatttagagcagcaacataaaactttattagaaagaaatactatatctggaccaaaaaactgcaacatggtttggaaatctaatgactaagaaggtaaaactggcaactatgtgcaactactgctcgtagatttgggtttgtttcccccccaacatctttaaaataagcagcccccacaaagggataatccattgaataaggagacaatgtagccaaagaagggatttgtggaaaaccatatgaatttaaatcaacataaaaagaacacacaaaggccatggaaacttgagaaggtgaaagaaaaaaaaaaaaaaccccaagcaaggacaagtcagctccttggagctgcaccaactcttaagtaggatgtccctattctaacggaaattgatgagtccacacctgggcacttcagtttgagaaatcaattggttggactggccattaaaaaaaggactttgtttttaaggtagataaagcttagagagagaaagctaaacagaaaagtaccaaatccttgtgaactcaaaaatgatttaggaagtcaaatgaagcaaactaaaaaactggatgaaaatgtttctctaagagtaaaacccagttttctctgtgatttaaaatcaaacaaacacactatagaagagaaattttcaaagtgcacccaataaaacctcagaggttccctggagtgtttggggtagcatggattgagacaggaagtgggttcaggcccatctcccccaacccttcttcactttaattcaaacatttctaattctcttttgtcgtttgtagtttcaggtaagatatcattttaaaaaaatgaaaaaaaaaaaaaatctaatgctgtccctttccctaagtttgaaaatcactgctgagactgaaattacattggtgagaaatatgatcatcataaatctaaaacacattttctatgtagtgctaccaaaatacaaagtttcatcaaatatttcactactattctgtaaaataaatgagaaaattaagttgttgggaagaaattaaattttgttattaccacctcccaaaatctgctcttctgctggctccaagatatcaatatttgatagtgtgaacaaatttctaacaaacattccagtcacaccgtaccccaaagacatttcattcaatggctgcatagtttcttttttgagaaggcaagcctcaaatttatagaaaactctagaatgaaaaatgtacaattactaaaaacataataacacactttatgtcagggcagaatctgcatagtgcttttaaacataatcaccaatgaagagtagccaaatcccagaacttcacacagcactcattagcaaacaacgtcaaagtgtaaatgataagcaggaaaaaaaccaagtaacacgaatgccatttttctttgatgcaatcacgaagaaaagtggaaatgcaggacgaaaagtggaatccaagctttggccacgtactgaaacttcattacttcaatgaaacagagcaaatctccatggaaaggactcattcagcaaacattaagttctttccatatattttttttccttcacgtaaggttaaacagaagttgctgtcattctagaatcagtgattacaattttttttttaattagaaaaaaggttacttgaatatttacataattttattgctctttattttaacaaaaacttttttcactgatttgtagactccatccattaacgtatgaaagtgaaatccatctctcaggaagatacagttatggttgaatgtatctgatgctgagagtacagcataattaagaaaaatccttgcatgtcatttggttcttgttgcagtcttctgtgttcacccctcagaaagcaaaagaatccatctgactttcaataaataccaaattattaaaaaaaaaaaaaaaagaacgtttccacagactagagatccaagaaaaagcagttctgatgaatgattcccagaatcaagtgagtcctcctttagtccaatgagatgatgtcaggaatgttacttccactgctggttatgacccctgtctcactcctgctgctggatgaactaacatgagtactgctttcatgggagctggtggtggtgacagacgtactgcttgctgttaagggtgaggtgagactatccaaaaacataggaggacagtactggggatcaactggaataagggaaagaaaatccaaacctggcaaatctgatgacatgcttgatattggcgtatggtggaatggtactgagtagtctgttaatgaaggcggaatagcagcaggatcaaccgaagtcacactgggcacccttacagaagatggctgatacatgagaacccctttggttgggctgctttgtgtttctgacataaagatgcatttccttttggcaggagggtcttcctcttcgtcagaagagctttctattgtaagatcaataacatctactttcttcttgcttgcctcactggctacagtcactgaacaaggcttactgaggacgcttgaactttctatttttgtacacggttggctggatactttcatagcttctttcttcggtctcattggacaccaagaaccatcttcttggaatttgatctcatctacatcagaacagtcattgagaatttccataaaaagcccatctaatattagactttcataggcagcttttttgtcacacacaggacaaatccaggtgggctttttctcattcatttgtagatagagggcagcatcaaaacactgcagatgtgtacaagtcactgcacggcatgggattgtcagcctcatttttcctaaagggcacatcaaggatacccgaaggctagttgtagcaatttcactatcaggatctgcagtaagtttttctttaattagtgctctggaatgatcagggtttctaatacctttcatttttaatctctgtaataacatggctgatgtaagctgccgtacaagatatacagacatagagtaattcttcccaatttctgatgcccaagaaatggaaatttggtttggcacagctgaagataacctaactaaagatgtaatattcaaggggcgtccagggcgcttctgttcaatcccatttttaggcggtggtgcatagccaggcaaaggaaatagcttcccatttacttttatacatagactatttggatagttatcttcttgagggcaacttgtctctgccaggcaaagtctcaactgaacttggactgtataatctctcctaccacctggcaaaaaatccctggatatgcatatctctctaacttgttgaggtgtcaaagcaaaaataaaaaacttctcttgaaatcgctgaatactgctttgaactaaactcgtgggcttgatgagaacatcaaggacatcataaaagggcagattttttaactgcacatcaggatggacaggaggaattgggggagatggctgctgcatctcaaatgtgggcttagtatcttgaagcagcacagaaccaacaggagaggatggtgagtgaggtgtaactgaagtggaaggcaacgagtggattccagccacggccaagtcaggttctacaggtgatgagccaccatccaaactgaaaaccgatgatttgattgtggataaatcagaaagtccttcaagagttcgtggatatcggcgtctatacaattctcggattttaatctgaaccgcagggctgcagccgctcttcaataaatgcagcgccctcatcaggaggtcatgcttgcgtccacttttattccgtccagcaaagcctagtaatacttgtagttcagaaaccctaaaactagaaaccatattcctcaactcttcgaaatccgccattttataccacccgcgggcgccgccgccgctgccgccgcacccactcccgctgccgccaacgacgctgccgccaccacggccgccgccgcctccagcaccatcctgcactgggcgccgcttaagacgccgcggccgccgccgctacagccgggcccgtcacgt

SEQ ID NO: 13723 - RNA, 8139 nt, Homo sapiens
  source 1..8139: mol_type = other RNA
gctgggattacaggcatgagccaccatgcccagcttaagaattcttgatttttggaaccttgattataagctgcctgatgtctggaaccaaaacttctgtaacactctattccacgtgtacttacaaaacactctaaacatttattaaacagtttgatgaaggccaaaataagaggcatatgctattctacaacacggtaacactcttcgtcacttaaaataattaagctttgagaacacaaaataaagctttttaaaaaagccattcagaaataggaagcagtttgggaaatgattgtgctacgccaatcaagaaaatgttgtacctcaaacatctgaaggtagcaatctgtttttttctttccctgcagctacccttattggaaacataagggaatataaagtgaaaacaggcaatgtttgcctgtttttatagcttttagccttaccacttttcagtttggggatggaatgcctttggctcagtagattctactggctttggggagctcagaaaggccataatggggcctacaggaagaggaaaaagagagctgacctcttaagggcaggccttaggtacaagaggctttttttaaaaagtgacaaaacttttgaactaaagatggaaaacgtagtctgacaaagaatatttgtgcaactttacagtgccagtaaaatcatgggaaaagcttggatagccatacgtaggtgtttctgaaacatgtcagattttatatatatatatatatatatatatatatttttttttttttttttttttttttttagagagtcttgctttgttacccaggctggagtgcagtggcacaatctcggatcactgcaaatcctccgcctcctgggttcaagcgattctcctgcctcggtctcccaagtagctgggactacaggcgcctgccatcacacccacctaatttatgtttttgctagagatggggtttcaccatgttccatgttagccaggctggtctccaactcctgacttcagattatctgcccgccttggcctcccaaagtgctgggattacaggcgtgagcctccatacccggcccatgtcagatatatttaaaactaagaaagcttgggaaaatctctgccaatgatctccatatcagttaaccccgttccatagagtcagaaaggcagagggtcttagtgcagatgcctgcataaagataaaacgttgcatgttcttggaaaatatggctagaccacccttcccataccatctagctgcagtataaattaacatacccatgtggaaaagtggtatgaatcaagaactacaaaagtgttcatatacccttgactagaaattccacctccagtattttatcctaagaaaataatttatacacaaagacattcattgtggcattatgagatataatctaaactgttcaaaataagtaaaggttatatgaaacatggcacatccataacaatggagtaccataaaattaataatagttgacacagttttaatgacatggaataatgcctgtaggttgcggggaaaaaccccaagatataaattacactgagaatgatgaaactaagtaaaaatatgcagaagtagcaaagacaatggcaaggaagatgcaaaaatatcaagtgattttttctggtgacagaatcataggcaattaattgttatacttttctgtattgtctaaattttccacaataagcatgtactactgacataaacagaaaaaacaaacattattcaaccaggcaagcattaaagaatggacattgggtacagctttatttatttcttttaggaattgcaggttcctaacaaagtaggggtgaggggggtgttacaaaccagtcactaggcaggaacattagactccaaaagcagagaaatgcttaattttcttctacctgtttcaccacattcatgtagaactgtagtaaaaaagatggtgaatcaggctgaatcaatctaaataacaacttaaggctcccaaatcacatgaacctaggaccactaaatccaatgtcagacgtgtttaaatggtgcactgctctacatttttctattatgcaaagagctagaaaataatggtagtgtcattatgacattccatgaaaatgaagaaaatctttcaggaaaaattaagaaaataaaaatgtttactaaagaaagaatggtccggctaagtgcttttttttttttttttttttttaaaccaactgaaggccagagaaatgaaaggcatacccgtgaattaaattaatgctttaaaaaaaattgactttacttaaaatacaaacaaacgtcaactaatgaatactttattggcagaaaaaaaagacaacttggctggaaatgctgagtgtcttggactggtctgaaggaagaacatctgaaaggtctgaatgtcaaagtcagaacagtctctggtcaatcctactttgcttaaaatccaacattttacctttcttcaaattcctcaagactaaggaaaacttggttttataccaagaattatgaatcaacctacacttgctatcccttacatcacattttcattctagcttttctgaaacacattaccagataaatgccatataacctaaattcacctcaatgctttcattttgcctttacaattaccttaggacagatgccaagtttttataacttcaggccagaaaatcctcaagtggctcacctaattgtcagaaagtgagtgagtgacaacagacctcaggcacgaaactattttcagcaccaattacactgtggggggttaccagaacaagaaaaggccttcatagttctaagtgaagaaagataaaaacattttattttggccaggcgcggtggctcacgcctgtaaatcccagcactttgggaggccaaggcaggcggatcacctgaggtcgggagttcgagaccagcctgaccaaaatggagaaaccccgtatctactaaaaatacaaaattagctgggcgtggtgatacatgcctgtaatcccagctactcgggaggctgaggcaggagaatcgcttgaaccctgtaggtggaggttgcggtgagccaagatcgcaccattgcactccatcccgggcaacaagagcaagactcagcctcaaaaaaaaaaaaaaaaaaattgattttaggaggctgacaattacagttcatttcctaagatattccagacaatcactggttggctgacagaatctaggtgacagctaagatcacccctctgaaactcccttatatttggttaagcagaaatctgggctagcaaaataaactactagaaagtcagggtctggataagaaacagtgaccacattaaaggctgacggattaataatcatgatgttgccataaggccaaagtcataaagtactaatgctcaagacagataaacaacgtaagccccaatttcaagatgataaacttcaaagtgtattttttaaaatgcaagttgcctgtatgaaataaattaaaaatttatatgtaatttcagtgtaaaacaccaaaaccgaacattaaaactgttcacagaaaatagaaaaaaaaacaaaaaaacaaatcacaattataaaagcacagagatatcagttataagaaccaagtaaataaactaatttctattaatattttcatttactttataaaactttgttgattaaattgggggagtctctgacaatctaaagggtaacaaaataacaaatatacatcatttctttataagtcataccacacaaaccaagttaagttttttctatctgattacagagtcaataaatattgcatctgtatttagagcagcaacataaaactttattagaaagaaatactatatctggaccaaaaaactgcaacatggtttggaaatctaatgactaagaaggtaaaactggcaactatgtgcaactactgctcgtagatttgggtttgtttcccccccaacatctttaaaataagcagcccccacaaagggataatccattgaataaggagacaatgtagccaaagaagggatttgtggaaaaccatatgaatttaaatcaacataaaaagaacacacaaaggccatggaaacttgagaaggtgaaagaaaaaaaaaaaaaaccccaagcaaggacaagtcagctccttggagctgcaccaactcttaagtaggatgtccctattctaacggaaattgatgagtccacacctgggcacttcagtttgagaaatcaattggttggactggccattaaaaaaaggactttgtttttaaggtagataaagcttagagagagaaagctaaacagaaaagtaccaaatccttgtgaactcaaaaatgatttaggaagtcaaatgaagcaaactaaaaaactggatgaaaatgtttctctaagagtaaaacccagttttctctgtgatttaaaatcaaacaaacacactatagaagagaaattttcaaagtgcacccaataaaacctcagaggttccctggagtgtttggggtagcatggattgagacaggaagtgggttcaggcccatctcccccaacccttcttcactttaattcaaacatttctaattctcttttgtcgtttgtagtttcaggtaagatatcattttaaaaaaatgaaaaaaaaaaaaaatctaatgctgtccctttccctaagtttgaaaatcactgctgagactgaaattacattggtgagaaatatgatcatcataaatctaaaacacattttctatgtagtgctaccaaaatacaaagtttcatcaaatatttcactactattctgtaaaataaatgagaaaattaagttgttgggaagaaattaaattttgttattaccacctcccaaaatctgctcttctgctggctccaagatatcaatatttgatagtgtgaacaaatttctaacaaacattccagtcacaccgtaccccaaagacatttcattcaatggctgcatagtttcttttttgagaaggcaagcctcaaatttatagaaaactctagaatgaaaaatgtacaattactaaaaacataataacacactttatgtcagggcagaatctgcatagtgcttttaaacataatcaccaatgaagagtagccaaatcccagaacttcacacagcactcattagcaaacaacgtcaaagtgtaaatgataagcaggaaaaaaaccaagtaacacgaatgccatttttctttgatgcaatcacgaagaaaagtggaaatgcaggacgaaaagtggaatccaagctttggccacgtactgaaacttcattacttcaatgaaacagagcaaatctccatggaaaggactcattcagcaaacattaagttctttccatatattttttttccttcacgtaaggttaaacagaagttgctgtcattctagaatcagtgattacaattttttttttaattagaaaaaaggttacttgaatatttacataattttattgctctttattttaacaaaaacttttttcactgatttgtagactccatccattaacgtatgaaagtgaaatccatctctcaggaagatacagttatggttgaatgtatctgatgctgagagtacagcataattaagaaaaatccttgcatgtcatttggttcttgttgcagtcttctgtgttcacccctcagaaagcaaaagaatccatctgactttcaataaataccaaattattaaaaaaaaaaaaaaaagaacgtttccacagactagagatccaagaaaaagcagttctgatgaatgattcccagaatcaagtgagtcctcctttagtccaatgagatgatgtcaggaatgttacttccactgctggttatgacccctgtctcactcctgctgctggatgaactaacatgagtactgctttcatgggagctggtggtggtgacagacgtactgcttgctgttaagggtgaggtgagactatccaaaaacataggaggacagtactggggatcaactggaataagggaaagaaaatccaaacctggcaaatctgatgacatgcttgatattggcgtatggtggaatggtactgagtagtctgttaatgaaggcggaatagcagcaggatcaaccgaagtcacactgggcacccttacagaagatggctgatacatgagaacccctttggttgggctgctttgtgtttctgacataaagatgcatttccttttggcaggagggtcttcctcttcgtcagaagagctttctattgtaagatcaataacatctactttcttcttgcttgcctcactggctacagtcactgaacaaggcttactgaggacgcttgaactttctatttttgtacacggttggctggatactttcatagcttctttcttcggtctcattggacaccaagaaccatcttcttggaatttgatctcatctacatcagaacagtcattgagaatttccataaaaagcccatctaatattagactttcataggcagcttttttgtcacacacaggacaaatccaggtgggctttttctcattcatttgtagatagagggcagcatcaaaacactgcagatgtgtacaagtcactgcacggcatgggattgtcagcctcatttttcctaaagggcacatcaaggatacccgaaggctagttgtagcaatttcactatcaggatctgcagtaagtttttctttaattagtgctctggaatgatcagggtttctaatacctttcatttttaatctctgtaataacatggctgatgtaagctgccgtacaagatatacagacatagagtaattcttcccaatttctgatgcccaagaaatggaaatttggtttggcacagctgaagataacctaactaaagatgtaatattcaaggggcgtccagggcgcttctgttcaatcccatttttaggcggtggtgcatagccaggcaaaggaaatagcttcccatttacttttatacatagactatttggatagttatcttcttgagggcaacttgtctctgccaggcaaagtctcaactgaacttggactgtataatctctcctaccacctggcaaaaaatccctggatatgcatatctctctaacttgttgaggtgtcaaagcaaaaataaaaaacttctcttgaaatcgctgaatactgctttgaactaaactcgtgggcttgatgagaacatcaaggacatcataaaagggcagattttttaactgcacatcaggatggacaggaggaattgggggagatggctgctgcatctcaaatgtgggcttagtatcttgaagcagcacagaaccaacaggagaggatggtgagtgaggtgtaactgaagtggaaggcaacgagtggattccagccacggccaagtcaggttctacaggtgatgagccaccatccaaactgaaaaccgatgatttgattgtggataaatcagaaagtccttcaagagttcgtggatatcggcgtctatacaattctcggattttaatctgaaccgcagggctgcagccgctcttcaataaatgcagcgccctcatcaggaggtcatgcttgcgtccacttttattccgtccagcaaagcctagtaatacttgtagttcagaaaccctaaaactagaaaccatattctaagcttgactctcagaggaatttctaggaggtctcatatctcatatttccagtgataacattatttggcaaaggatgttaatgcaactggctctatgggcagaatggctaaaatgaaaaacactgataacaccaaatgctggcgaggatgctgagaaactggatcactccatacattgctggtagggatgtaaaatggtacagccacttgtgaaactttgaaagcattccctttaaaatcaggaacaagatcaggatgcccccatcacagcttctattcaacattgtactggagatccctcaactcttcgaaatccgccattttataccacccgcgggcgccgccgccgctgccgccgcacccactcccgctgccgccaacgacgctgccgccaccacggccgccgccgcctccagcaccatcctgcactgggcgccgcttaagacgccgcggccgccgccgctacagccgggcccgtcacgt

SEQ ID NO: 13724 - RNA, 8161 nt, Homo sapiens
  source 1..8161: mol_type = other RNA
gctgggattacaggcatgagccaccatgcccagcttaagaattcttgatttttggaaccttgattataagctgcctgatgtctggaaccaaaacttctgtaacactctattccacgtgtacttacaaaacactctaaacatttattaaacagtttgatgaaggccaaaataagaggcatatgctattctacaacacggtaacactcttcgtcacttaaaataattaagctttgagaacacaaaataaagctttttaaaaaagccattcagaaataggaagcagtttgggaaatgattgtgctacgccaatcaagaaaatgttgtacctcaaacatctgaaggtagcaatctgtttttttctttccctgcagctacccttattggaaacataagggaatataaagtgaaaacaggcaatgtttgcctgtttttatagcttttagccttaccacttttcagtttggggatggaatgcctttggctcagtagattctactggctttggggagctcagaaaggccataatggggcctacaggaagaggaaaaagagagctgacctcttaagggcaggccttaggtacaagaggctttttttaaaaagtgacaaaacttttgaactaaagatggaaaacgtagtctgacaaagaatatttgtgcaactttacagtgccagtaaaatcatgggaaaagcttggatagccatacgtaggtgtttctgaaacatgtcagattttatatatatatatatatatatatatatatttttttttttttttttttttttttttagagagtcttgctttgttacccaggctggagtgcagtggcacaatctcggatcactgcaaatcctccgcctcctgggttcaagcgattctcctgcctcggtctcccaagtagctgggactacaggcgcctgccatcacacccacctaatttatgtttttgctagagatggggtttcaccatgttccatgttagccaggctggtctccaactcctgacttcagattatctgcccgccttggcctcccaaagtgctgggattacaggcgtgagcctccatacccggcccatgtcagatatatttaaaactaagaaagcttgggaaaatctctgccaatgatctccatatcagttaaccccgttccatagagtcagaaaggcagagggtcttagtgcagatgcctgcataaagataaaacgttgcatgttcttggaaaatatggctagaccacccttcccataccatctagctgcagtataaattaacatacccatgtggaaaagtggtatgaatcaagaactacaaaagtgttcatatacccttgactagaaattccacctccagtattttatcctaagaaaataatttatacacaaagacattcattgtggcattatgagatataatctaaactgttcaaaataagtaaaggttatatgaaacatggcacatccataacaatggagtaccataaaattaataatagttgacacagttttaatgacatggaataatgcctgtaggttgcggggaaaaaccccaagatataaattacactgagaatgatgaaactaagtaaaaatatgcagaagtagcaaagacaatggcaaggaagatgcaaaaatatcaagtgattttttctggtgacagaatcataggcaattaattgttatacttttctgtattgtctaaattttccacaataagcatgtactactgacataaacagaaaaaacaaacattattcaaccaggcaagcattaaagaatggacattgggtacagctttatttatttcttttaggaattgcaggttcctaacaaagtaggggtgaggggggtgttacaaaccagtcactaggcaggaacattagactccaaaagcagagaaatgcttaattttcttctacctgtttcaccacattcatgtagaactgtagtaaaaaagatggtgaatcaggctgaatcaatctaaataacaacttaaggctcccaaatcacatgaacctaggaccactaaatccaatgtcagacgtgtttaaatggtgcactgctctacatttttctattatgcaaagagctagaaaataatggtagtgtcattatgacattccatgaaaatgaagaaaatctttcaggaaaaattaagaaaataaaaatgtttactaaagaaagaatggtccggctaagtgcttttttttttttttttttttttaaaccaactgaaggccagagaaatgaaaggcatacccgtgaattaaattaatgctttaaaaaaaattgactttacttaaaatacaaacaaacgtcaactaatgaatactttattggcagaaaaaaaagacaacttggctggaaatgctgagtgtcttggactggtctgaaggaagaacatctgaaaggtctgaatgtcaaagtcagaacagtctctggtcaatcctactttgcttaaaatccaacattttacctttcttcaaattcctcaagactaaggaaaacttggttttataccaagaattatgaatcaacctacacttgctatcccttacatcacattttcattctagcttttctgaaacacattaccagataaatgccatataacctaaattcacctcaatgctttcattttgcctttacaattaccttaggacagatgccaagtttttataacttcaggccagaaaatcctcaagtggctcacctaattgtcagaaagtgagtgagtgacaacagacctcaggcacgaaactattttcagcaccaattacactgtggggggttaccagaacaagaaaaggccttcatagttctaagtgaagaaagataaaaacattttattttggccaggcgcggtggctcacgcctgtaaatcccagcactttgggaggccaaggcaggcggatcacctgaggtcgggagttcgagaccagcctgaccaaaatggagaaaccccgtatctactaaaaatacaaaattagctgggcgtggtgatacatgcctgtaatcccagctactcgggaggctgaggcaggagaatcgcttgaaccctgtaggtggaggttgcggtgagccaagatcgcaccattgcactccatcccgggcaacaagagcaagactcagcctcaaaaaaaaaaaaaaaaaaattgattttaggaggctgacaattacagttcatttcctaagatattccagacaatcactggttggctgacagaatctaggtgacagctaagatcacccctctgaaactcccttatatttggttaagcagaaatctgggctagcaaaataaactactagaaagtcagggtctggataagaaacagtgaccacattaaaggctgacggattaataatcatgatgttgccataaggccaaagtcataaagtactaatgctcaagacagataaacaacgtaagccccaatttcaagatgataaacttcaaagtgtattttttaaaatgcaagttgcctgtatgaaataaattaaaaatttatatgtaatttcagtgtaaaacaccaaaaccgaacattaaaactgttcacagaaaatagaaaaaaaaacaaaaaaacaaatcacaattataaaagcacagagatatcagttataagaaccaagtaaataaactaatttctattaatattttcatttactttataaaactttgttgattaaattgggggagtctctgacaatctaaagggtaacaaaataacaaatatacatcatttctttataagtcataccacacaaaccaagttaagttttttctatctgattacagagtcaataaatattgcatctgtatttagagcagcaacataaaactttattagaaagaaatactatatctggaccaaaaaactgcaacatggtttggaaatctaatgactaagaaggtaaaactggcaactatgtgcaactactgctcgtagatttgggtttgtttcccccccaacatctttaaaataagcagcccccacaaagggataatccattgaataaggagacaatgtagccaaagaagggatttgtggaaaaccatatgaatttaaatcaacataaaaagaacacacaaaggccatggaaacttgagaaggtgaaagaaaaaaaaaaaaaaccccaagcaaggacaagtcagctccttggagctgcaccaactcttaagtaggatgtccctattctaacggaaattgatgagtccacacctgggcacttcagtttgagaaatcaattggttggactggccattaaaaaaaggactttgtttttaaggtagataaagcttagagagagaaagctaaacagaaaagtaccaaatccttgtgaactcaaaaatgatttaggaagtcaaatgaagcaaactaaaaaactggatgaaaatgtttctctaagagtaaaacccagttttctctgtgatttaaaatcaaacaaacacactatagaagagaaattttcaaagtgcacccaataaaacctcagaggttccctggagtgtttggggtagcatggattgagacaggaagtgggttcaggcccatctcccccaacccttcttcactttaattcaaacatttctaattctcttttgtcgtttgtagtttcaggtaagatatcattttaaaaaaatgaaaaaaaaaaaaaatctaatgctgtccctttccctaagtttgaaaatcactgctgagactgaaattacattggtgagaaatatgatcatcataaatctaaaacacattttctatgtagtgctaccaaaatacaaagtttcatcaaatatttcactactattctgtaaaataaatgagaaaattaagttgttgggaagaaattaaattttgttattaccacctcccaaaatctgctcttctgctggctccaagatatcaatatttgatagtgtgaacaaatttctaacaaacattccagtcacaccgtaccccaaagacatttcattcaatggctgcatagtttcttttttgagaaggcaagcctcaaatttatagaaaactctagaatgaaaaatgtacaattactaaaaacataataacacactttatgtcagggcagaatctgcatagtgcttttaaacataatcaccaatgaagagtagccaaatcccagaacttcacacagcactcattagcaaacaacgtcaaagtgtaaatgataagcaggaaaaaaaccaagtaacacgaatgccatttttctttgatgcaatcacgaagaaaagtggaaatgcaggacgaaaagtggaatccaagctttggccacgtactgaaacttcattacttcaatgaaacagagcaaatctccatggaaaggactcattcagcaaacattaagttctttccatatattttttttccttcacgtaaggttaaacagaagttgctgtcattctagaatcagtgattacaattttttttttaattagaaaaaaggttacttgaatatttacataattttattgctctttattttaacaaaaacttttttcactgatttgtagactccatccattaacgtatgaaagtgaaatccatctctcaggaagatacagttatggttgaatgtatctgatgctgagagtacagcataattaagaaaaatccttgcatgtcatttggttcttgttgcagtcttctgtgttcacccctcagaaagcaaaagaatccatctgactttcaataaataccaaattattaaaaaaaaaaaaaaaagaacgtttccacagactagagatccaagaaaaagcagttctgatgaatgattcccagaatcaagtgagtcctcctttagtccaatgagatgatgtcaggaatgttacttccactgctggttatgacccctgtctcactcctgctgctggatgaactaacatgagtactgctttcatgggagctggtggtggtgacagacgtactgcttgctgttaagggtgaggtgagactatccaaaaacataggaggacagtactggggatcaactggaataagggaaagaaaatccaaacctggcaaatctgatgacatgcttgatattggcgtatggtggaatggtactgagtagtctgttaatgaaggcggaatagcagcaggatcaaccgaagtcacactgggcacccttacagaagatggctgatacatgagaacccctttggttgggctgctttgtgtttctgacataaagatgcatttccttttggcaggagggtcttcctcttcgtcagaagagctttctattgtaagatcaataacatctactttcttcttgcttgcctcactggctacagtcactgaacaaggcttactgaggacgcttgaactttctatttttgtacacggttggctggatactttcatagcttctttcttcggtctcattggacaccaagaaccatcttcttggaatttgatctcatctacatcagaacagtcattgagaatttccataaaaagcccatctaatattagactttcataggcagcttttttgtcacacacaggacaaatccaggtgggctttttctcattcatttgtagatagagggcagcatcaaaacactgcagatgtgtacaagtcactgcacggcatgggattgtcagcctcatttttcctaaagggcacatcaaggatacccgaaggctagttgtagcaatttcactatcaggatctgcagtaagtttttctttaattagtgctctggaatgatcagggtttctaatacctttcatttttaatctctgtaataacatggctgatgtaagctgccgtacaagatatacagacatagagtaattcttcccaatttctgatgcccaagaaatggaaatttggtttggcacagctgaagataacctaactaaagatgtaatattcaaggggcgtccagggcgcttctgttcaatcccatttttaggcggtggtgcatagccaggcaaaggaaatagcttcccatttacttttatacatagactatttggatagttatcttcttgagggcaacttgtctctgccaggcaaagtctcaactgaacttggactgtataatctctcctaccacctggcaaaaaatccctggatatgcatatctctctaacttgttgaggtgtcaaagcaaaaataaaaaacttctcttgaaatcgctgaatactgctttgaactaaactcgtgggcttgatgagaacatcaaggacatcataaaagggcagattttttaactgcacatcaggatggacaggaggaattgggggagatggctgctgcatctcaaatgtgggcttagtatcttgaagcagcacagaaccaacaggagaggatggtgagtgaggtgtaactgaagtggaaggcaacgagtggattccagccacggccaagtcaggttctacaggtgatgagccaccatccaaactgaaaaccgatgatttgattgtggataaatcagaaagtccttcaagagttcgtggatatcggcgtctatacaattctcggattttaatctgaaccgcagggctgcagccgctcttcaataaatgcagcgccctcatcaggaggtcatgcttgcgtccacttttattccgtccagcaaagcctagtaatacttgtagttcagaaaccctaaaactagaaaccatattctgtaatcccagctactcgggaggttgaggtaggagaattgcttgaacccgggaggcacaggttgcagcgagccgagatcgtgccattgcactccagcctgggcaacaaaagtaaaactctgtcagaatggctaaaatgaaaaacactgataacaccaaatgctggcgaggatgctgagaaactggatcactccatacattgctggtagggatgtaaaatggtacagccacttgtgaaactttgaaagcattccctttaaaatcaggaacaagatcaggatgcccccatcacagcttctattcaacattgtactggagatccctcaactcttcgaaatccgccattttataccacccgcgggcgccgccgccgctgccgccgcacccactcccgctgccgccaacgacgctgccgccaccacggccgccgccgcctccagcaccatcctgcactgggcgccgcttaagacgccgcggccgccgccgctacagccgggcccgtcacgt

SEQ ID NO: 13725 - RNA, 8012 nt, Homo sapiens
  source 1..8012: mol_type = other RNA
gctgggattacaggcatgagccaccatgcccagcttaagaattcttgatttttggaaccttgattataagctgcctgatgtctggaaccaaaacttctgtaacactctattccacgtgtacttacaaaacactctaaacatttattaaacagtttgatgaaggccaaaataagaggcatatgctattctacaacacggtaacactcttcgtcacttaaaataattaagctttgagaacacaaaataaagctttttaaaaaagccattcagaaataggaagcagtttgggaaatgattgtgctacgccaatcaagaaaatgttgtacctcaaacatctgaaggtagcaatctgtttttttctttccctgcagctacccttattggaaacataagggaatataaagtgaaaacaggcaatgtttgcctgtttttatagcttttagccttaccacttttcagtttggggatggaatgcctttggctcagtagattctactggctttggggagctcagaaaggccataatggggcctacaggaagaggaaaaagagagctgacctcttaagggcaggccttaggtacaagaggctttttttaaaaagtgacaaaacttttgaactaaagatggaaaacgtagtctgacaaagaatatttgtgcaactttacagtgccagtaaaatcatgggaaaagcttggatagccatacgtaggtgtttctgaaacatgtcagattttatatatatatatatatatatatatatatttttttttttttttttttttttttttagagagtcttgctttgttacccaggctggagtgcagtggcacaatctcggatcactgcaaatcctccgcctcctgggttcaagcgattctcctgcctcggtctcccaagtagctgggactacaggcgcctgccatcacacccacctaatttatgtttttgctagagatggggtttcaccatgttccatgttagccaggctggtctccaactcctgacttcagattatctgcccgccttggcctcccaaagtgctgggattacaggcgtgagcctccatacccggcccatgtcagatatatttaaaactaagaaagcttgggaaaatctctgccaatgatctccatatcagttaaccccgttccatagagtcagaaaggcagagggtcttagtgcagatgcctgcataaagataaaacgttgcatgttcttggaaaatatggctagaccacccttcccataccatctagctgcagtataaattaacatacccatgtggaaaagtggtatgaatcaagaactacaaaagtgttcatatacccttgactagaaattccacctccagtattttatcctaagaaaataatttatacacaaagacattcattgtggcattatgagatataatctaaactgttcaaaataagtaaaggttatatgaaacatggcacatccataacaatggagtaccataaaattaataatagttgacacagttttaatgacatggaataatgcctgtaggttgcggggaaaaaccccaagatataaattacactgagaatgatgaaactaagtaaaaatatgcagaagtagcaaagacaatggcaaggaagatgcaaaaatatcaagtgattttttctggtgacagaatcataggcaattaattgttatacttttctgtattgtctaaattttccacaataagcatgtactactgacataaacagaaaaaacaaacattattcaaccaggcaagcattaaagaatggacattgggtacagctttatttatttcttttaggaattgcaggttcctaacaaagtaggggtgaggggggtgttacaaaccagtcactaggcaggaacattagactccaaaagcagagaaatgcttaattttcttctacctgtttcaccacattcatgtagaactgtagtaaaaaagatggtgaatcaggctgaatcaatctaaataacaacttaaggctcccaaatcacatgaacctaggaccactaaatccaatgtcagacgtgtttaaatggtgcactgctctacatttttctattatgcaaagagctagaaaataatggtagtgtcattatgacattccatgaaaatgaagaaaatctttcaggaaaaattaagaaaataaaaatgtttactaaagaaagaatggtccggctaagtgcttttttttttttttttttttttaaaccaactgaaggccagagaaatgaaaggcatacccgtgaattaaattaatgctttaaaaaaaattgactttacttaaaatacaaacaaacgtcaactaatgaatactttattggcagaaaaaaaagacaacttggctggaaatgctgagtgtcttggactggtctgaaggaagaacatctgaaaggtctgaatgtcaaagtcagaacagtctctggtcaatcctactttgcttaaaatccaacattttacctttcttcaaattcctcaagactaaggaaaacttggttttataccaagaattatgaatcaacctacacttgctatcccttacatcacattttcattctagcttttctgaaacacattaccagataaatgccatataacctaaattcacctcaatgctttcattttgcctttacaattaccttaggacagatgccaagtttttataacttcaggccagaaaatcctcaagtggctcacctaattgtcagaaagtgagtgagtgacaacagacctcaggcacgaaactattttcagcaccaattacactgtggggggttaccagaacaagaaaaggccttcatagttctaagtgaagaaagataaaaacattttattttggccaggcgcggtggctcacgcctgtaaatcccagcactttgggaggccaaggcaggcggatcacctgaggtcgggagttcgagaccagcctgaccaaaatggagaaaccccgtatctactaaaaatacaaaattagctgggcgtggtgatacatgcctgtaatcccagctactcgggaggctgaggcaggagaatcgcttgaaccctgtaggtggaggttgcggtgagccaagatcgcaccattgcactccatcccgggcaacaagagcaagactcagcctcaaaaaaaaaaaaaaaaaaattgattttaggaggctgacaattacagttcatttcctaagatattccagacaatcactggttggctgacagaatctaggtgacagctaagatcacccctctgaaactcccttatatttggttaagcagaaatctgggctagcaaaataaactactagaaagtcagggtctggataagaaacagtgaccacattaaaggctgacggattaataatcatgatgttgccataaggccaaagtcataaagtactaatgctcaagacagataaacaacgtaagccccaatttcaagatgataaacttcaaagtgtattttttaaaatgcaagttgcctgtatgaaataaattaaaaatttatatgtaatttcagtgtaaaacaccaaaaccgaacattaaaactgttcacagaaaatagaaaaaaaaacaaaaaaacaaatcacaattataaaagcacagagatatcagttataagaaccaagtaaataaactaatttctattaatattttcatttactttataaaactttgttgattaaattgggggagtctctgacaatctaaagggtaacaaaataacaaatatacatcatttctttataagtcataccacacaaaccaagttaagttttttctatctgattacagagtcaataaatattgcatctgtatttagagcagcaacataaaactttattagaaagaaatactatatctggaccaaaaaactgcaacatggtttggaaatctaatgactaagaaggtaaaactggcaactatgtgcaactactgctcgtagatttgggtttgtttcccccccaacatctttaaaataagcagcccccacaaagggataatccattgaataaggagacaatgtagccaaagaagggatttgtggaaaaccatatgaatttaaatcaacataaaaagaacacacaaaggccatggaaacttgagaaggtgaaagaaaaaaaaaaaaaaccccaagcaaggacaagtcagctccttggagctgcaccaactcttaagtaggatgtccctattctaacggaaattgatgagtccacacctgggcacttcagtttgagaaatcaattggttggactggccattaaaaaaaggactttgtttttaaggtagataaagcttagagagagaaagctaaacagaaaagtaccaaatccttgtgaactcaaaaatgatttaggaagtcaaatgaagcaaactaaaaaactggatgaaaatgtttctctaagagtaaaacccagttttctctgtgatttaaaatcaaacaaacacactatagaagagaaattttcaaagtgcacccaataaaacctcagaggttccctggagtgtttggggtagcatggattgagacaggaagtgggttcaggcccatctcccccaacccttcttcactttaattcaaacatttctaattctcttttgtcgtttgtagtttcaggtaagatatcattttaaaaaaatgaaaaaaaaaaaaaatctaatgctgtccctttccctaagtttgaaaatcactgctgagactgaaattacattggtgagaaatatgatcatcataaatctaaaacacattttctatgtagtgctaccaaaatacaaagtttcatcaaatatttcactactattctgtaaaataaatgagaaaattaagttgttgggaagaaattaaattttgttattaccacctcccaaaatctgctcttctgctggctccaagatatcaatatttgatagtgtgaacaaatttctaacaaacattccagtcacaccgtaccccaaagacatttcattcaatggctgcatagtttcttttttgagaaggcaagcctcaaatttatagaaaactctagaatgaaaaatgtacaattactaaaaacataataacacactttatgtcagggcagaatctgcatagtgcttttaaacataatcaccaatgaagagtagccaaatcccagaacttcacacagcactcattagcaaacaacgtcaaagtgtaaatgataagcaggaaaaaaaccaagtaacacgaatgccatttttctttgatgcaatcacgaagaaaagtggaaatgcaggacgaaaagtggaatccaagctttggccacgtactgaaacttcattacttcaatgaaacagagcaaatctccatggaaaggactcattcagcaaacattaagttctttccatatattttttttccttcacgtaaggttaaacagaagttgctgtcattctagaatcagtgattacaattttttttttaattagaaaaaaggttacttgaatatttacataattttattgctctttattttaacaaaaacttttttcactgatttgtagactccatccattaacgtatgaaagtgaaatccatctctcaggaagatacagttatggttgaatgtatctgatgctgagagtacagcataattaagaaaaatccttgcatgtcatttggttcttgttgcagtcttctgtgttcacccctcagaaagcaaaagaatccatctgactttcaataaataccaaattattaaaaaaaaaaaaaaaagaacgtttccacagactagagatccaagaaaaagcagttctgatgaatgattcccagaatcaagtgagtcctcctttagtccaatgagatgatgtcaggaatgttacttccactgctggttatgacccctgtctcactcctgctgctggatgaactaacatgagtactgctttcatgggagctggtggtggtgacagacgtactgcttgctgttaagggtgaggtgagactggggatcaactggaataagggaaagaaaatccaaacctggcaaatctgatgacatgcttgatattggcgtatggtggaatggtactgagtagtctgttaatgaaggcggaatagcagcaggatcaaccgaagtcacactgggcacccttacagaagatggctgatacatgagaacccctttggttgggctgctttgtgtttctgacataaagatgcatttccttttggcaggagggtcttcctcttcgtcagaagagctttctattgtaagatcaataacatctactttcttcttgcttgcctcactggctacagtcactgaacaaggcttactgaggacgcttgaactttctatttttgtacacggttggctggatactttcatagcttctttcttcggtctcattggacaccaagaaccatcttcttggaatttgatctcatctacatcagaacagtcattgagaatttccataaaaagcccatctaatattagactttcataggcagcttttttgtcacacacaggacaaatccaggtgggctttttctcattcatttgtagatagagggcagcatcaaaacactgcagatgtgtacaagtcactgcacggcatgggattgtcagcctcatttttcctaaagggcacatcaaggatacccgaaggctagttgtagcaatttcactatcaggatctgcagtaagtttttctttaattagtgctctggaatgatcagggtttctaatacctttcatttttaatctctgtaataacatggctgatgtaagctgccgtacaagatatacagacatagagtaattcttcccaatttctgatgcccaagaaatggaaatttggtttggcacagctgaagataacctaactaaagatgtaatattcaaggggcgtccagggcgcttctgttcaatcccatttttaggcggtggtgcatagccaggcaaaggaaatagcttcccatttacttttatacatagactatttggatagttatcttcttgagggcaacttgtctctgccaggcaaagtctcaactgaacttggactgtataatctctcctaccacctggcaaaaaatccctggatatgcatatctctctaacttgttgaggtgtcaaagcaaaaataaaaaacttctcttgaaatcgctgaatactgctttgaactaaactcgtgggcttgatgagaacatcaaggacatcataaaagggcagattttttaactgcacatcaggatggacaggaggaattgggggagatggctgctgcatctcaaatgtgggcttagtatcttgaagcagcacagaaccaacaggagaggatggtgagtgaggtgtaactgaagtggaaggcaacgagtggattccagccacggccaagtcaggttctacaggtgatgagccaccatccaaactgaaaaccgatgatttgattgtggataaatcagaaagtccttcaagagttcgtggatatcggcgtctatacaattctcggattttaatctgaaccgcagggctgcagccgctcttcaataaatgcagcgccctcatcaggaggtcatgcttgcgtccacttttattccgtccagcaaagcctagtaatacttgtagttcagaaaccctaaaactagaaaccatattcagaatggctaaaatgaaaaacactgataacaccaaatgctggcgaggatgctgagaaactggatcactccatacattgctggtagggatgtaaaatggtacagccacttgtgaaactttgaaagcattccctttaaaatcaggaacaagatcaggatgcccccatcacagcttctattcaacattgtactggagatccctcaactcttcgaaatccgccattttataccacccgcgggcgccgccgccgctgccgccgcacccactcccgctgccgccaacgacgctgccgccaccacggccgccgccgcctccagcaccatcctgcactgggcgccgcttaagacgccgcggccgccgccgctacagccgggcccgtcacgt

SEQ ID NO: 13726 - RNA, 833 nt, Homo sapiens
  source 1..833: mol_type = other RNA
gctgggattacaggcatgagccaccatgcccaggcaagactccttgtaatggtaaagttgtaattactatatcaacgagcaataagactattacatgagggacctggagaagtcaaatacacagggacagaaagtagaacggtgactgccaggggcacggggaggaagaacagggagttgtttaacagggacagagtatcagttttgcaagatgaaaagctttctggagattggctgcacaccagtgtgactatccttaacactactgaatcgtatacttaaatataataaagaagataaatttcatgttatgtgtattttaccacaataaagagaaaaaagaaagaaaaaagagcaacaagcctacccaacctgtcaaacaggaagggatatacgatatccacggccactgtactgtgtcctaggcatttttgcatctgaaatctcatttagcttcccgacatgctttctagggaagtgtgtttccatcaaacaaacaaggaaagtcagactcagcgaaatcatggacttgacctaaggtcattcacttggtccctggtagagccaagactcatgtacttgttatgttttgttccttatactatagctaattaccctcccactcaggctattacaaaaaaaaaaagaaagaaagagagaaagattacactgcatgttttttccattacatgtttaataatttaaagttctccatgataacctcaggcaaactagaattaatcttcaaaatcaggttagtgcaaaaagaaaacatttctagtttgttcctgaaacacattcatcctattcgatatgcaccttaccttttaatc

SEQ ID NO: 13727 - RNA, 1724 nt, Homo sapiens
  source 1..1724: mol_type = other RNA
gctgggattacaggcatgagccaccatgcccaggcaggaatgtagacaattttcttgtataacacagtttctaccagtcacattgcttgatccttcgtctctccacctgagtccttgcaaccaaggttgcatgaaaaaattgaagggtgatgaatgcggagaattttattactgatgaaagtggctcccagcaggatggggagctggaagggggatggagtgggaaggtgatcttcccatggagtccagcagtcccctgctgtacacttctcctaagtcccaccatcaagccattcctctgaagtcaagctgtttctttccaatgtctggctacttcttctcttctctccttctttgccatctttgtaaaagaggcccaagggagcttgttcactccttccatcatgtgaagaagcagcaagaatgcaccacctatgaagctgagaacacgccttcatctgaatctgctggtacgttgatcttggacttcccaggctccagaacctgatgccttactgaagagagcaccagctttcctgtcagaagccatcttcaccttcgcaagtgtttttttgtttgtttgttttttgttttttttgtttgtttgtttgtttttcagacagggctttatgagcaaaaaagctgtatgtgtgtgaggggagaatgtggcatgagacagtttttcttctggagacaaggaactctgttctggtgagcttcctgctgtgctctaaggaccttcaagttgccagaggatttttagcatggactgggccccatgaatgtccggtgacaataaagatattcctggataaacatttcttttttttctttccaccagggccctgtccatgctaacttcttttaaacttttcaaaccgattgatggtaaagcatacatcaagtcatattcagtttaatagacatttagcgggtgcctactatgtgtaaggccctgtggatgcaaagcagaagaatatacagagatctctgcagaaagactgcgggggcttctgtagcatctccattctcagccacccaatcctacccaaccacagtatctcttgggagcagatgctgctgatgtgggcagagcagagttagcaaaggcacgacttgtcacacaccactgccacaatccgtggctgtaagagggcctcagcgacctttttgggcgtgggctgtttggttcagcttcctcttctgagaccccatctcctagctgcatatcatgctagcaggacccagagagatttatctggtgacctttctgcatgcggaatccaagcagggggaccgagaaaatcagctccgaagcggttaattttactggctcctaaattgataagcggtggtacgtcagtctgaaatgaactcgccttgttcgacggggttctaagacagcggaactcaatcaacagcgggccgcaaggttcaaggctgcaattcatcccgccgtgcctctgaaaaatgggaggtgacagttcattttgccagtgacagtctgtcggtctcgctcgctgcttctcctgtcgattgcctggctgaggtgaagtgcagctcagaaacaccctcgtttggtattctactcagctgagcaggatggtcccaggacccaaggtgtgcaaatcttactgcccctacagcttgtcttcttcccttctgggaagctctgaactgctcatgcatgattatgggtcccaggagtcatcttcccacttcct

SEQ ID NO: 13728 - RNA, 534 nt, Homo sapiens
  source 1..534: mol_type = other RNA
gctgggattacaggcatgagccaccatgcccagtcgatatctcactttttattttgccatggatgagagtcctgggtgtgaggaacacctcccaccaggctagaggcaactgcccaggaaggactgtgcttccgtcacctctaaatcccttgcagatccttgataaatgcctcatgaagaccaatctcttgaatcccatatctacccagaattaactccattccagtctctgcatgtaatcagttttatccacagaaacattttcattttaggaaatccctggttttaagtatcaatccttgttcagctggacaatatgaatcttttccactgaagttagggatgactgtgattttcagaacacgtccagaatttttcatcaagaaggtagcttgagcctgagatcaggagtttgagaccagcctgggcaacatggtgaaatcccgtctctactaaaaacacaaaaactagccgggcatggtggctggcgcctgtaatcccagctactcaggaggctgaggcaggagaatcact

SEQ ID NO: 13729 - RNA, 3897 nt, Homo sapiens
  source 1..3897: mol_type = other RNA
gctgggattacaggcatgagccaccatgcccagtctatttttattttttgagacaggatctggctctattgcccagggtggagtgcaatagtgcaatcttggctcactgcagcctctgcctcccaggctcaaaccatcctcccacctcagcctcctgagtagctaggactacaggcgtgtaccaacatgcccatctaatttttgtatttttggtagagatggggtttcgccatgttgcccagactggtctggaactcctgggctcaagtgaacctcccaccttggcctcccaaagtgctgggattacagacgtgagccaccatacccatccctattttctttaaaaaatgtgttttttacaaaatgtatggtaagtatatgtatttactgtgctttgtgataattttctcagtgacaaaaaatttccaattttgttaacatccatggtaaaatgatctaatttcaaaaatttgttctagagccaagatccttataacctctataaatgtgtgtgaatagttagttggcaggtcctacaaagaaatgtcatttttattcatgtattttgggttgtttaaacatttctgtaagatttaaaatacttttcttcttatggctagaattctcagcatctactcccatgcctgcctttctaaaatctattggccagtttaagggtatttacaataatacaacttaaagacaaagtgtccataagtcattatttctaacagacagcataacacagtagaaattgccctgaccaaggaattagaagactggaattcaagtcctaactctgccactaactttgcaggatgaccttaggcaagtcatgtcacttctctcatttgtcaaataatgcaaatgattccattctaaggtattttccacctctaaaattgctttcatttactattattattttttaaataatgaaaacactttctgggaattgtcttaagcccaaatgggtagagaagaattttttttttttttttttttttttgagacagagtctcgctctgtcgcctaggctggagtgcagtggtgcaatctcggcttactgcaccctctgcctcccgggttcaagtgattctcttgcctcagcctcctgggtagctgggattacaggtgagcaccaccacgcccggctaatttttgtatttttagtagagatggcgtttcaccatgttggtcaggctggtctcgaactcctgaccttgtgatccacccacctcggcctcccaaagtgctgggattacaggcatgagccactgcgcctggccgagtagagaagaatttactgctgattaaggttgtgtttttcaacctgcaatcccgagaccctcagaataaagattacttgaggttgctatgaaaaatacagattcctgtcctccccctggctgaatcagaatctcataaggtgaggctcaggtttctgcacttttcacaagctctgtaatggttacagtgcaccctaatgtttgagaaccagtggcctaaagagaatgcaacctaagagggcaaggctagtgcatagcttaaatcgctccagcctttggtaatcccttctaaacacagtaccacccatgtggaggagactgcaaggaagctgttattcaaagtagaacagtcagccttgtgcttgagtcctgctttatgcttgcgtgtttcataacaaaacacaaaggcaagtcttcatatcagcacttagtcttgatatccaagtagctgactactgtacttatgataacagcttgaagaggactgcaactctcccctcacgaatggtgacagagttggcttgtcacacctggctcagggaagaaaaatgagtaaacccctacctctttactcttgattcctcttccaccctaatactgttaacacatcatcctgtgtgattcaaataatctggcagatgaaatacagaaaatctaagtcatattgttcttatcactctatggccagatattatactaatctaattttaaaaatccttttctgtgcaatagaaataaccaaagctcattctgtctcctttcctttctaatgctgttgataggaacaaaatatcaagtaaggatacatgctagagatgttaaattcatacaagtaaagtaaattacaaagagaggtggtaatatttttttctagaatttcacaataaaatccctctcaccatgaaaatctttttataattttaacaggaaacttaaaagacattttgttgcaagactatcttaacaattataagaataatgccattatctgtgctcaatatagataaacataacagtaactttaaaaggccaagtatactcataagtgaggatgaaatttatttttcaacaaccaatatgccaatatccaacttctaggttttattcaattctaatgtcatgggtttctcctaccccagtcaaaactcctgccaaatgtccacaaaattgacaccaaaatcaacaaacacaaagaaagagagggacagggagagggaaagagaaatagagagtgaggaaggaaggaacgtgacaagagctaccatgcaaaatgaccagaagaactggagttcagtggcacagatcagcaggagcagaggaatgctgcaaaagatgatgctgcatagagtctaacttggagatgcctgtatgatgctggatgaccaagtactaaggtcacaagtgtgttcatggacccataagaaccaggatcttgacccaaacttataagatcttctaaaaagaaaatacttcatctaaattgaagcaattcctaagtcaaacaccagaagagttccttatttgatgtaagttgtgcctaaaactttggctgatacaaagaaacccgtccactaaggcaccctgaggcaatctgacaatgtgttggagagaactttgttgtcagtaccacatcattatgagagtacagagaacggatcacccgcaggggactggcttctttgggcaagcagtcaacaagttcactgcactgtttgtcaaatcccaacaagcgaatcccatagccatgtggggaagaaatcattcgtccatcggggctgaagcaaagttctttgatgtaacccctgcctacattggcttcttcaatgtaatgagtcagtcgtagagaacagcgaggtgagacaggtcgcactggagctccttcttggaattcatagacacaagtacactcctcatcatcactgttgcttgagcaccgaagaagagtggcccagccttttgggtgcagctgtaaggacgtgatgcagtttccgtggtcactctcaccaagaacttcaggggttacgacttcaagactatttcgtggtgaaactccttctctttgagaggctcgtgacatgtgtttctcagaagaattagaatcactatgatgacaaggtgagccagaaactctaggaccagatgaacttgatgaagtggtcaaatctgaacttgaagtagttcttcttgctcttaaaatgggatagctgcctacttctaaagacttagttaagtcaaggtcatgcaaaattaagagatatccagaggacgttgaaatcaacattttggaacaatctggtgttaacctcattcgcatgagaaaacgtgtgtgaaagaatttcttatgtggacacccatcttctgtatacctgatattatttacacagtcttcatgagcttcagaaagtgtttttatgtgctttgaagatatagggtcaaaaagcagaacttcagtttgttcacaagcaactgtcagcactgactgtgtaccagaaagccctagttgtgggctggctctgacaggtccgctgtgtagcttcgggcatttctccttcacagagcccaagtcctgaaggcgagcaagtggggccccgcctgcctgcctcaaaaa

SEQ ID NO: 13730 - RNA, 4576 nt, Homo sapiens
  source 1..4576: mol_type = other RNA
gctgggattacaggcatgagccaccatgcccagtctatttttattttttgagacaggatctggctctattgcccagggtggagtgcaatagtgcaatcttggctcactgcagcctctgcctcccaggctcaaaccatcctcccacctcagcctcctgagtagctaggactacaggcgtgtaccaacatgcccatctaatttttgtatttttggtagagatggggtttcgccatgttgcccagactggtctggaactcctgggctcaagtgaacctcccaccttggcctcccaaagtgctgggattacagacgtgagccaccatacccatccctattttctttaaaaaatgtgttttttacaaaatgtatggtaagtatatgtatttactgtgctttgtgataattttctcagtgacaaaaaatttccaattttgttaacatccatggtaaaatgatctaatttcaaaaatttgttctagagccaagatccttataacctctataaatgtgtgtgaatagttagttggcaggtcctacaaagaaatgtcatttttattcatgtattttgggttgtttaaacatttctgtaagatttaaaatacttttcttcttatggctagaattctcagcatctactcccatgcctgcctttctaaaatctattggccagtttaagggtatttacaataatacaacttaaagacaaagtgtccataagtcattatttctaacagacagcataacacagtagaaattgccctgaccaaggaattagaagactggaattcaagtcctaactctgccactaactttgcaggatgaccttaggcaagtcatgtcacttctctcatttgtcaaataatgcaaatgattccattctaaggtattttccacctctaaaattgctttcatttactattattattttttaaataatgaaaacactttctgggaattgtcttaagcccaaatgggtagagaagaattttttttttttttttttttttttgagacagagtctcgctctgtcgcctaggctggagtgcagtggtgcaatctcggcttactgcaccctctgcctcccgggttcaagtgattctcttgcctcagcctcctgggtagctgggattacaggtgagcaccaccacgcccggctaatttttgtatttttagtagagatggcgtttcaccatgttggtcaggctggtctcgaactcctgaccttgtgatccacccacctcggcctcccaaagtgctgggattacaggcatgagccactgcgcctggccgagtagagaagaatttactgctgattaaggttgtgtttttcaacctgcaatcccgagaccctcagaataaagattacttgaggttgctatgaaaaatacagattcctgtcctccccctggctgaatcagaatctcataaggtgaggctcaggtttctgcacttttcacaagctctgtaatggttacagtgcaccctaatgtttgagaaccagtggcctaaagagaatgcaacctaagagggcaaggctagtgcatagcttaaatcgctccagcctttggtaatcccttctaaacacagtaccacccatgtggaggagactgcaaggaagctgttattcaaagtagaacagtcagccttgtgcttgagtcctgctttatgcttgcgtgtttcataacaaaacacaaaggcaagtcttcatatcagcacttagtcttgatatccaagtagctgactactgtacttatgataacagcttgaagaggactgcaactctcccctcacgaatggtgacagagttggcttgtcacacctggctcagggaagaaaaatgagtaaacccctacctctttactcttgattcctcttccaccctaatactgttaacacatcatcctgtgtgattcaaataatctggcagatgaaatacagaaaatctaagtcatattgttcttatcactctatggccagatattatactaatctaattttaaaaatccttttctgtgcaatagaaataaccaaagctcattctgtctcctttcctttctaatgctgttgataggaacaaaatatcaagtaaggatacatgctagagatgttaaattcatacaagtaaagtaaattacaaagagaggtggtaatatttttttctagaatttcacaataaaatccctctcaccatgaaaatctttttataattttaacaggaaacttaaaagacattttgttgcaagactatcttaacaattataagaataatgccattatctgtgctcaatatagataaacataacagtaactttaaaaggccaagtatactcataagtgaggatgaaatttatttttcaacaaccaatatgccaatatccaacttctaggttttattcaattctaatgtcatgggtttctcctaccccagtcaaaactcctgccaaatgtccacaaaattgacaccaaaatcaacaaacacaaagaaagagagggacagggagagggaaagagaaatagagagtgaggaaggaaggaacgtgacaagagctaccatgcaaaatgaccagaagaactggagttcagtggcacagatcagcaggagcagaggaatgctgcaaaagatgatgctgcatagagtctaacttggagatgcctgtatgatgctggatgaccaagtactaaggtcacaagtgtgttcatggacccataagaaccaggatcttgacccaaacttataagatcttctaaaaagaaaatacttcatctaaattgaagcaattcctaagtcaaacaccagaagagttccttatttgatgtaagttgtgcctaaaactttggctgatacaaagaaacccgtccactaaggcaccctgaggcaatctgacaatgtgttggagagaactttgttgtcagtaccacatcattatgagagtacagagaacggatcacccgcaggggactggcttctttgggcaagcagtcaacaagttcactgcactgtttgtcaaatcccaacaagcgaatcccatagccatgtggggaagaaatcattcgtccatcggggctgaagcaaagttctttgatgtaacccctgcctacattggcttcttcaatgtaatgagtcagtcgtagagaacagcgaggtgagacaggtcgcactggagctccttcttggaattcatagacacaagtacactcctcatcatcactgttgcttgagcaccgaagaagagtggcccagccttttgggtgcagctgtaaggacgtgatgcagtttccgtggtcactctcaccaagaacttcaggggttacgacttcaagactatttcgtggtgaaactccttctctttgagaggctcgtgacatgtgtttctcagaagaattagaatcactatgatgacaaggtgagccagaaactctaggaccagatgaacttgatgaagtggtcaaatctgaacttgaagtagttcttcttgctcttaaaatgggatagctgcctacttctaaagacttagttaagtcaaggtcatgcaaaattaagagatatccagaggacgttgaaatcaacattttggaacaatctggtgttaacctcattcgcatgagaaaacgtgtgtgaaagaatttcttatgtggacacccatcttctgtatacctgttagtgtcccaaataatgacatttccatcaaatcctgatgttactaagagtcttgtattagtatcatattcgatgttcttcacccagctagtgtgaccatgtaaagtgcatactttggtgttcaattttctcagatcccatagtgctattgtagtgtcatcagagcaggtagcaaacagccggttatcaagaaatctgatattatttacacagtcttcatgagcttcagaaagtgtttttatgtgctttgaagatatagggtcaaaaagcagaacttcagtttgttcacaagcaactgtcagcactgacccgtcgggcgagtactcgaggttgaagacggcgccgtgggtgcgggtgctgaggtacaccgagtccgcggggtggatggaaccgtagaggctagtcatggtgcgaaaattgtcccgcgccgggtccacgaacagcccgcggcccaggctgcgctctttcagccacccgaacagcctagcgccagggccgcccaggcccgcgccgaggccgtgtcggccccggctcttggccctgcagtctggcccgggccgccggcacggaggggagggaggtgacggctctcccggggcggaggcagttgaggactccggagctccaggcagccctagctctccggagcgcggggccggggacagcgatggggcgccggggcggcgagggcttcgggcgggtggagggggatgggtcgcatcagccccgggatgtagtggcgagggcggcccggtggctgctgcctgcccctcgtggggcgtcggctcctcagccccggctccggccgatccgtcccctccagggctatggggcccaaagggaaacatgatcaacgcccccgccccccgctccgggccactgccccgccggccgacacctcagtgcccctgttcagct

SEQ ID NO: 13731 - RNA, 4061 nt, Homo sapiens
  source 1..4061: mol_type = other RNA
gctgggattacaggcatgagccaccatgcccagtctatttttattttttgagacaggatctggctctattgcccagggtggagtgcaatagtgcaatcttggctcactgcagcctctgcctcccaggctcaaaccatcctcccacctcagcctcctgagtagctaggactacaggcgtgtaccaacatgcccatctaatttttgtatttttggtagagatggggtttcgccatgttgcccagactggtctggaactcctgggctcaagtgaacctcccaccttggcctcccaaagtgctgggattacagacgtgagccaccatacccatccctattttctttaaaaaatgtgttttttacaaaatgtatggtaagtatatgtatttactgtgctttgtgataattttctcagtgacaaaaaatttccaattttgttaacatccatggtaaaatgatctaatttcaaaaatttgttctagagccaagatccttataacctctataaatgtgtgtgaatagttagttggcaggtcctacaaagaaatgtcatttttattcatgtattttgggttgtttaaacatttctgtaagatttaaaatacttttcttcttatggctagaattctcagcatctactcccatgcctgcctttctaaaatctattggccagtttaagggtatttacaataatacaacttaaagacaaagtgtccataagtcattatttctaacagacagcataacacagtagaaattgccctgaccaaggaattagaagactggaattcaagtcctaactctgccactaactttgcaggatgaccttaggcaagtcatgtcacttctctcatttgtcaaataatgcaaatgattccattctaaggtattttccacctctaaaattgctttcatttactattattattttttaaataatgaaaacactttctgggaattgtcttaagcccaaatgggtagagaagaattttttttttttttttttttttttgagacagagtctcgctctgtcgcctaggctggagtgcagtggtgcaatctcggcttactgcaccctctgcctcccgggttcaagtgattctcttgcctcagcctcctgggtagctgggattacaggtgagcaccaccacgcccggctaatttttgtatttttagtagagatggcgtttcaccatgttggtcaggctggtctcgaactcctgaccttgtgatccacccacctcggcctcccaaagtgctgggattacaggcatgagccactgcgcctggccgagtagagaagaatttactgctgattaaggttgtgtttttcaacctgcaatcccgagaccctcagaataaagattacttgaggttgctatgaaaaatacagattcctgtcctccccctggctgaatcagaatctcataaggtgaggctcaggtttctgcacttttcacaagctctgtaatggttacagtgcaccctaatgtttgagaaccagtggcctaaagagaatgcaacctaagagggcaaggctagtgcatagcttaaatcgctccagcctttggtaatcccttctaaacacagtaccacccatgtggaggagactgcaaggaagctgttattcaaagtagaacagtcagccttgtgcttgagtcctgctttatgcttgcgtgtttcataacaaaacacaaaggcaagtcttcatatcagcacttagtcttgatatccaagtagctgactactgtacttatgataacagcttgaagaggactgcaactctcccctcacgaatggtgacagagttggcttgtcacacctggctcagggaagaaaaatgagtaaacccctacctctttactcttgattcctcttccaccctaatactgttaacacatcatcctgtgtgattcaaataatctggcagatgaaatacagaaaatctaagtcatattgttcttatcactctatggccagatattatactaatctaattttaaaaatccttttctgtgcaatagaaataaccaaagctcattctgtctcctttcctttctaatgctgttgataggaacaaaatatcaagtaaggatacatgctagagatgttaaattcatacaagtaaagtaaattacaaagagaggtggtaatatttttttctagaatttcacaataaaatccctctcaccatgaaaatctttttataattttaacaggaaacttaaaagacattttgttgcaagactatcttaacaattataagaataatgccattatctgtgctcaatatagataaacataacagtaactttaaaaggccaagtatactcataagtgaggatgaaatttatttttcaacaaccaatatgccaatatccaacttctaggttttattcaattctaatgtcatgggtttctcctaccccagtcaaaactcctgccaaatgtccacaaaattgacaccaaaatcaacaaacacaaagaaagagagggacagggagagggaaagagaaatagagagtgaggaaggaaggaacgtgacaagagctaccatgcaaaatgaccagaagaactggagttcagtggcacagatcagcaggagcagaggaatgctgcaaaagatgatgctgcatagagtctaacttggagatgcctgtatgatgctggatgaccaagtactaaggtcacaagtgtgttcatggacccataagaaccaggatcttgacccaaacttataagatcttctaaaaagaaaatacttcatctaaattgaagcaattcctaagtcaaacaccagaagagttccttatttgatgtaagttgtgcctaaaactttggctgatacaaagaaacccgtccactaaggcaccctgaggcaatctgacaatgtgttggagagaactttgttgtcagtaccacatcattatgagagtacagagaacggatcacccgcaggggactggcttctttgggcaagcagtcaacaagttcactgcactgtttgtcaaatcccaacaagcgaatcccatagccatgtggggaagaaatcattcgtccatcggggctgaagcaaagttctttgatgtaacccctgcctacattggcttcttcaatgtaatgagtcagtcgtagagaacagcgaggtgagacaggtcgcactggagctccttcttggaattcatagacacaagtacactcctcatcatcactgttgcttgagcaccgaagaagagtggcccagccttttgggtgcagctgtaaggacgtgatgcagtttccgtggtcactctcaccaagaacttcaggggttacgacttcaagactatttcgtggtgaaactccttctctttgagaggctcgtgacatgtgtttctcagaagaattagaatcactatgatgacaaggtgagccagaaactctaggaccagatgaacttgatgaagtggtcaaatctgaacttgaagtagttcttcttgctcttaaaatgggatagctgcctacttctaaagacttagttaagtcaaggtcatgcaaaattaagagatatccagaggacgttgaaatcaacattttggaacaatctggtgttaacctcattcgcatgagaaaacgtgtgtgaaagaatttcttatgtggacacccatcttctgtatacctgttagtgtcccaaataatgacatttccatcaaatcctgatgttactaagagtcttgtattagtatcatattcgatgttcttcacccagctagtgtgaccatgtaaagtgcatactttggtgttcaattttctcagatcccatagtgctattgtagtgtcatcagagcaggtagcaaacagccggttatcaagaaatctgatattatttacacagtcttcatgagcttcagaaagtgtttttatgtgctttgaagatatagggtcaaaaagcagaacttcagtttgttcacaagcaactgtcagcactgacctgtgtgagcgactgagcatctgggcacctgatctgggtggcagagtcggtctgtagttgtcagtgaccggtggccgcgtgcctggggatgagt

SEQ ID NO: 13732 - RNA, 4781 nt, Homo sapiens
  source 1..4781: mol_type = other RNA
gctgggattacaggcatgagccaccatgcccagtctatttttattttttgagacaggatctggctctattgcccagggtggagtgcaatagtgcaatcttggctcactgcagcctctgcctcccaggctcaaaccatcctcccacctcagcctcctgagtagctaggactacaggcgtgtaccaacatgcccatctaatttttgtatttttggtagagatggggtttcgccatgttgcccagactggtctggaactcctgggctcaagtgaacctcccaccttggcctcccaaagtgctgggattacagacgtgagccaccatacccatccctattttctttaaaaaatgtgttttttacaaaatgtatggtaagtatatgtatttactgtgctttgtgataattttctcagtgacaaaaaatttccaattttgttaacatccatggtaaaatgatctaatttcaaaaatttgttctagagccaagatccttataacctctataaatgtgtgtgaatagttagttggcaggtcctacaaagaaatgtcatttttattcatgtattttgggttgtttaaacatttctgtaagatttaaaatacttttcttcttatggctagaattctcagcatctactcccatgcctgcctttctaaaatctattggccagtttaagggtatttacaataatacaacttaaagacaaagtgtccataagtcattatttctaacagacagcataacacagtagaaattgccctgaccaaggaattagaagactggaattcaagtcctaactctgccactaactttgcaggatgaccttaggcaagtcatgtcacttctctcatttgtcaaataatgcaaatgattccattctaaggtattttccacctctaaaattgctttcatttactattattattttttaaataatgaaaacactttctgggaattgtcttaagcccaaatgggtagagaagaattttttttttttttttttttttttgagacagagtctcgctctgtcgcctaggctggagtgcagtggtgcaatctcggcttactgcaccctctgcctcccgggttcaagtgattctcttgcctcagcctcctgggtagctgggattacaggtgagcaccaccacgcccggctaatttttgtatttttagtagagatggcgtttcaccatgttggtcaggctggtctcgaactcctgaccttgtgatccacccacctcggcctcccaaagtgctgggattacaggcatgagccactgcgcctggccgagtagagaagaatttactgctgattaaggttgtgtttttcaacctgcaatcccgagaccctcagaataaagattacttgaggttgctatgaaaaatacagattcctgtcctccccctggctgaatcagaatctcataaggtgaggctcaggtttctgcacttttcacaagctctgtaatggttacagtgcaccctaatgtttgagaaccagtggcctaaagagaatgcaacctaagagggcaaggctagtgcatagcttaaatcgctccagcctttggtaatcccttctaaacacagtaccacccatgtggaggagactgcaaggaagctgttattcaaagtagaacagtcagccttgtgcttgagtcctgctttatgcttgcgtgtttcataacaaaacacaaaggcaagtcttcatatcagcacttagtcttgatatccaagtagctgactactgtacttatgataacagcttgaagaggactgcaactctcccctcacgaatggtgacagagttggcttgtcacacctggctcagggaagaaaaatgagtaaacccctacctctttactcttgattcctcttccaccctaatactgttaacacatcatcctgtgtgattcaaataatctggcagatgaaatacagaaaatctaagtcatattgttcttatcactctatggccagatattatactaatctaattttaaaaatccttttctgtgcaatagaaataaccaaagctcattctgtctcctttcctttctaatgctgttgataggaacaaaatatcaagtaaggatacatgctagagatgttaaattcatacaagtaaagtaaattacaaagagaggtggtaatatttttttctagaatttcacaataaaatccctctcaccatgaaaatctttttataattttaacaggaaacttaaaagacattttgttgcaagactatcttaacaattataagaataatgccattatctgtgctcaatatagataaacataacagtaactttaaaaggccaagtatactcataagtgaggatgaaatttatttttcaacaaccaatatgccaatatccaacttctaggttttattcaattctaatgtcatgggtttctcctaccccagtcaaaactcctgccaaatgtccacaaaattgacaccaaaatcaacaaacacaaagaaagagagggacagggagagggaaagagaaatagagagtgaggaaggaaggaacgtgacaagagctaccatgcaaaatgaccagaagaactggagttcagtggcacagatcagcaggagcagaggaatgctgcaaaagatgatgctgcatagagtctaacttggagatgcctgtatgatgctggatgaccaagtactaaggtcacaagtgtgttcatggacccataagaaccaggatcttgacccaaacttataagatcttctaaaaagaaaatacttcatctaaattgaagcaattcctaagtcaaacaccagaagagttccttatttgatgtaagttgtgcctaaaactttggctgatacaaagaaacccgtccactaaggcaccctgaggcaatctgacaatgtgttggagagaactttgttgtcagtaccacatcattatgagagtacagagaacggatcacccgcaggggactggcttctttgggcaagcagtcaacaagttcactgcactgtttgtcaaatcccaacaagcgaatcccatagccatgtggggaagaaatcattcgtccatcggggctgaagcaaagttctttgatgtaacccctgcctacattggcttcttcaatgtaatgagtcagtcgtagagaacagcgaggtgagacaggtcgcactggagctccttcttggaattcatagacacaagtacactcttcccctacacaattcaaaggctcttctcttctctcctttcagttgtggcctctaggaccagtgagatccttggaagactcttgctttccagagtgatgagaatcataaagtcatttaacacctttccccctagtcatcagtatagtcccttcctttcccagagtttcccctcctcatcatcactgttgcttgagcaccgaagaagagtggcccagccttttgggtgcagctgtaaggacgtgatgcagtttccgtggtcactctcaccaagaacttcaggggttacgacttcaagactatttcgtggtgaaactccttctctttgagaggctcgtgacatgtgtttctcagaagaattagaatcactatgatgacaaggtgagccagaaactctaggaccagatgaacttgatgaagtggtcaaatctgaacttgaagtagttcttcttgctcttaaaatgggatagctgcctacttctaaagacttagttaagtcaaggtcatgcaaaattaagagatatccagaggacgttgaaatcaacattttggaacaatctggtgttaacctcattcgcatgagaaaacgtgtgtgaaagaatttcttatgtggacacccatcttctgtatacctgttagtgtcccaaataatgacatttccatcaaatcctgatgttactaagagtcttgtattagtatcatattcgatgttcttcacccagctagtgtgaccatgtaaagtgcatactttggtgttcaattttctcagatcccatagtgctattgtagtgtcatcagagcaggtagcaaacagccggttatcaagaaatctgatattatttacacagtcttcatgagcttcagaaagtgtttttatgtgctttgaagatatagggtcaaaaagcagaacttcagtttgttcacaagcaactgtcagcactgacccgtcgggcgagtactcgaggttgaagacggcgccgtgggtgcgggtgctgaggtacaccgagtccgcggggtggatggaaccgtagaggctagtcatggtgcgaaaattgtcccgcgccgggtccacgaacagcccgcggcccaggctgcgctctttcagccacccgaacagcctagcgccagggccgcccaggcccgcgccgaggccgtgtcggccccggctcttggccctgcagtctggcccgggccgccggcacggaggggagggaggtgacggctctcccggggcggaggcagttgaggactccggagctccaggcagccctagctctccggagcgcggggccggggacagcgatggggcgccggggcggcgagggcttcgggcgggtggagggggatgggtcgcatcagccccgggatgtagtggcgagggcggcccggtggctgctgcctgcccctcgtggggcgtcggctcctcagccccggctccggccgatccgtcccctccagggctatggggcccaaagggaaacatgatcaacgcccccgccccccgctccgggccactgccccgccggccgacacctcagtgcccctgttcagctgccacttccggcgtgcagcggcctaaccccac

SEQ ID NO: 13733 - RNA, 4906 nt, Homo sapiens
  source 1..4906: mol_type = other RNA
gctgggattacaggcatgagccaccatgcccagtctatttttattttttgagacaggatctggctctattgcccagggtggagtgcaatagtgcaatcttggctcactgcagcctctgcctcccaggctcaaaccatcctcccacctcagcctcctgagtagctaggactacaggcgtgtaccaacatgcccatctaatttttgtatttttggtagagatggggtttcgccatgttgcccagactggtctggaactcctgggctcaagtgaacctcccaccttggcctcccaaagtgctgggattacagacgtgagccaccatacccatccctattttctttaaaaaatgtgttttttacaaaatgtatggtaagtatatgtatttactgtgctttgtgataattttctcagtgacaaaaaatttccaattttgttaacatccatggtaaaatgatctaatttcaaaaatttgttctagagccaagatccttataacctctataaatgtgtgtgaatagttagttggcaggtcctacaaagaaatgtcatttttattcatgtattttgggttgtttaaacatttctgtaagatttaaaatacttttcttcttatggctagaattctcagcatctactcccatgcctgcctttctaaaatctattggccagtttaagggtatttacaataatacaacttaaagacaaagtgtccataagtcattatttctaacagacagcataacacagtagaaattgccctgaccaaggaattagaagactggaattcaagtcctaactctgccactaactttgcaggatgaccttaggcaagtcatgtcacttctctcatttgtcaaataatgcaaatgattccattctaaggtattttccacctctaaaattgctttcatttactattattattttttaaataatgaaaacactttctgggaattgtcttaagcccaaatgggtagagaagaattttttttttttttttttttttttgagacagagtctcgctctgtcgcctaggctggagtgcagtggtgcaatctcggcttactgcaccctctgcctcccgggttcaagtgattctcttgcctcagcctcctgggtagctgggattacaggtgagcaccaccacgcccggctaatttttgtatttttagtagagatggcgtttcaccatgttggtcaggctggtctcgaactcctgaccttgtgatccacccacctcggcctcccaaagtgctgggattacaggcatgagccactgcgcctggccgagtagagaagaatttactgctgattaaggttgtgtttttcaacctgcaatcccgagaccctcagaataaagattacttgaggttgctatgaaaaatacagattcctgtcctccccctggctgaatcagaatctcataaggtgaggctcaggtttctgcacttttcacaagctctgtaatggttacagtgcaccctaatgtttgagaaccagtggcctaaagagaatgcaacctaagagggcaaggctagtgcatagcttaaatcgctccagcctttggtaatcccttctaaacacagtaccacccatgtggaggagactgcaaggaagctgttattcaaagtagaacagtcagccttgtgcttgagtcctgctttatgcttgcgtgtttcataacaaaacacaaaggcaagtcttcatatcagcacttagtcttgatatccaagtagctgactactgtacttatgataacagcttgaagaggactgcaactctcccctcacgaatggtgacagagttggcttgtcacacctggctcagggaagaaaaatgagtaaacccctacctctttactcttgattcctcttccaccctaatactgttaacacatcatcctgtgtgattcaaataatctggcagatgaaatacagaaaatctaagtcatattgttcttatcactctatggccagatattatactaatctaattttaaaaatccttttctgtgcaatagaaataaccaaagctcattctgtctcctttcctttctaatgctgttgataggaacaaaatatcaagtaaggatacatgctagagatgttaaattcatacaagtaaagtaaattacaaagagaggtggtaatatttttttctagaatttcacaataaaatccctctcaccatgaaaatctttttataattttaacaggaaacttaaaagacattttgttgcaagactatcttaacaattataagaataatgccattatctgtgctcaatatagataaacataacagtaactttaaaaggccaagtatactcataagtgaggatgaaatttatttttcaacaaccaatatgccaatatccaacttctaggttttattcaattctaatgtcatgggtttctcctaccccagtcaaaactcctgccaaatgtccacaaaattgacaccaaaatcaacaaacacaaagaaagagagggacagggagagggaaagagaaatagagagtgaggaaggaaggaacgtgacaagagctaccatgcaaaatgaccagaagaactggagttcagtggcacagatcagcaggagcagaggaatgctgcaaaagatgatgctgcatagagtctaacttggagatgcctgtatgatgctggatgaccaagtactaaggtcacaagtgtgttcatggacccataagaaccaggatcttgacccaaacttataagatcttctaaaaagaaaatacttcatctaaattgaagcaattcctaagtcaaacaccagaagagttccttatttgatgtaagttgtgcctaaaactttggctgatacaaagaaacccgtccactaaggcaccctgaggcaatctgacaatgtgttggagagaactttgttgtcagtaccacatcattatgagagtacagagaacggatcacccgcaggggactggcttctttgggcaagcagtcaacaagttcactgcactgtttgtcaaatcccaacaagcgaatcccatagccatgtggggaagaaatcattcgtccatcggggctgaagcaaagttctttgatgtaacccctgcctacattggcttcttcaatgtaatgagtcagtcgtagagaacagcgaggtgagacaggtcgcactggagctccttcttggaattcatagacacaagtacactcttcccctacacaattcaaaggctcttctcttctctcctttcagttgtggcctctaggaccagtgagatccttggaagactcttgctttccagagtgatgagaatcataaagtcatttaacacctttccccctagtcatcagtatagtcccttcctttcccagagtttcccctggtttttaaaaaaagaaaattatgatactcaattggcttagtaaaatctcacatttagccagcttagctgaaacatttcagacctatgtttattatacaaggggtttttgtttgtttgtttgtttgtttgtttagggtgagatgaaagaggcaagatttaagaagctgggcaaaaactgagctgatgctggcctttaaagtacctcccaccttgctcaaccccagcaggagaggaataagaagagtttggaagggataatgataccatatgaagcaagagaggacagaaacaggagagtcgagaagcaggatctctagcagtatgcccttgaaggcagagactgcagtcagcgatcggcctaagctctgcacacacggcaatggcaatttgtccaatgagccctgttgaaggtggagtgctgctgcctgtacctcctcatcatcactgttgcttgagcaccgaagaagagtggcccagccttttgggtgcagctgtaaggacgtgatgcagtttccgtggtcactctcaccaagaacttcaggggttacgacttcaagactatttcgtggtgaaactcctgaacttgaagtagttcttcttgctcttaaaatgggatagctgcctacttctaaagacttagttaagtcaaggtcatgcaaaattaagagatatccagaggacgttgaaatcaacattttggaacaatctggtgttaacctcattcgcatgagaaaacgtgtgtgaaagaatttcttatgtggacacccatcttctgtatacctgatattatttacacagtcttcatgagcttcagaaagtgtttttatgtgctttgaagatatagggtcaaaaagcagaacttcagtttgttcacaagcaactgtcagcactgacccgtcgggcgagtactcgaggttgaagacggcgccgtgggtgcgggtgctgaggtacaccgagtccgcggggtggatggaaccgtagaggctagtcatggtgcgaaaattgtcccgcgccgggtccacgaacagcccgcggcccaggctgcgctctttcagccacccgaacagcctagcgccagggccgcccaggcccgcgccgaggccgtgtcggccccggctcttggccctgcagtctggcccgggccgccggcacggaggggagggaggtgacggctctcccggggcggaggcagttgaggactccggagctccaggcagccctagctctccggagcgcggggccggggacagcgatggggcgccggggcggcgagggcttcgggcgggtggagggggatgggtcgcatcagccccgggatgtagtggcgagggcggcccggtggctgctgcctgcccctcgtggggcgtcggctcctcagccccggctccggccgatccgtcccctccagggctatggggcccaaagggaaacatgatcaacgcccccgccccccgctccgggccactgccccgccggccgacacctcagtgcccctgttcagctgccacttccggcgtgcagcggcctaaccccac

SEQ ID NO: 13734 - RNA, 5104 nt, Homo sapiens
  source 1..5104: mol_type = other RNA
gctgggattacaggcatgagccaccatgcccagtctatttttattttttgagacaggatctggctctattgcccagggtggagtgcaatagtgcaatcttggctcactgcagcctctgcctcccaggctcaaaccatcctcccacctcagcctcctgagtagctaggactacaggcgtgtaccaacatgcccatctaatttttgtatttttggtagagatggggtttcgccatgttgcccagactggtctggaactcctgggctcaagtgaacctcccaccttggcctcccaaagtgctgggattacagacgtgagccaccatacccatccctattttctttaaaaaatgtgttttttacaaaatgtatggtaagtatatgtatttactgtgctttgtgataattttctcagtgacaaaaaatttccaattttgttaacatccatggtaaaatgatctaatttcaaaaatttgttctagagccaagatccttataacctctataaatgtgtgtgaatagttagttggcaggtcctacaaagaaatgtcatttttattcatgtattttgggttgtttaaacatttctgtaagatttaaaatacttttcttcttatggctagaattctcagcatctactcccatgcctgcctttctaaaatctattggccagtttaagggtatttacaataatacaacttaaagacaaagtgtccataagtcattatttctaacagacagcataacacagtagaaattgccctgaccaaggaattagaagactggaattcaagtcctaactctgccactaactttgcaggatgaccttaggcaagtcatgtcacttctctcatttgtcaaataatgcaaatgattccattctaaggtattttccacctctaaaattgctttcatttactattattattttttaaataatgaaaacactttctgggaattgtcttaagcccaaatgggtagagaagaattttttttttttttttttttttttgagacagagtctcgctctgtcgcctaggctggagtgcagtggtgcaatctcggcttactgcaccctctgcctcccgggttcaagtgattctcttgcctcagcctcctgggtagctgggattacaggtgagcaccaccacgcccggctaatttttgtatttttagtagagatggcgtttcaccatgttggtcaggctggtctcgaactcctgaccttgtgatccacccacctcggcctcccaaagtgctgggattacaggcatgagccactgcgcctggccgagtagagaagaatttactgctgattaaggttgtgtttttcaacctgcaatcccgagaccctcagaataaagattacttgaggttgctatgaaaaatacagattcctgtcctccccctggctgaatcagaatctcataaggtgaggctcaggtttctgcacttttcacaagctctgtaatggttacagtgcaccctaatgtttgagaaccagtggcctaaagagaatgcaacctaagagggcaaggctagtgcatagcttaaatcgctccagcctttggtaatcccttctaaacacagtaccacccatgtggaggagactgcaaggaagctgttattcaaagtagaacagtcagccttgtgcttgagtcctgctttatgcttgcgtgtttcataacaaaacacaaaggcaagtcttcatatcagcacttagtcttgatatccaagtagctgactactgtacttatgataacagcttgaagaggactgcaactctcccctcacgaatggtgacagagttggcttgtcacacctggctcagggaagaaaaatgagtaaacccctacctctttactcttgattcctcttccaccctaatactgttaacacatcatcctgtgtgattcaaataatctggcagatgaaatacagaaaatctaagtcatattgttcttatcactctatggccagatattatactaatctaattttaaaaatccttttctgtgcaatagaaataaccaaagctcattctgtctcctttcctttctaatgctgttgataggaacaaaatatcaagtaaggatacatgctagagatgttaaattcatacaagtaaagtaaattacaaagagaggtggtaatatttttttctagaatttcacaataaaatccctctcaccatgaaaatctttttataattttaacaggaaacttaaaagacattttgttgcaagactatcttaacaattataagaataatgccattatctgtgctcaatatagataaacataacagtaactttaaaaggccaagtatactcataagtgaggatgaaatttatttttcaacaaccaatatgccaatatccaacttctaggttttattcaattctaatgtcatgggtttctcctaccccagtcaaaactcctgccaaatgtccacaaaattgacaccaaaatcaacaaacacaaagaaagagagggacagggagagggaaagagaaatagagagtgaggaaggaaggaacgtgacaagagctaccatgcaaaatgaccagaagaactggagttcagtggcacagatcagcaggagcagaggaatgctgcaaaagatgatgctgcatagagtctaacttggagatgcctgtatgatgctggatgaccaagtactaaggtcacaagtgtgttcatggacccataagaaccaggatcttgacccaaacttataagatcttctaaaaagaaaatacttcatctaaattgaagcaattcctaagtcaaacaccagaagagttccttatttgatgtaagttgtgcctaaaactttggctgatacaaagaaacccgtccactaaggcaccctgaggcaatctgacaatgtgttggagagaactttgttgtcagtaccacatcattatgagagtacagagaacggatcacccgcaggggactggcttctttgggcaagcagtcaacaagttcactgcactgtttgtcaaatcccaacaagcgaatcccatagccatgtggggaagaaatcattcgtccatcggggctgaagcaaagttctttgatgtaacccctgcctacattggcttcttcaatgtaatgagtcagtcgtagagaacagcgaggtgagacaggtcgcactggagctccttcttggaattcatagacacaagtacactcttcccctacacaattcaaaggctcttctcttctctcctttcagttgtggcctctaggaccagtgagatccttggaagactcttgctttccagagtgatgagaatcataaagtcatttaacacctttccccctagtcatcagtatagtcccttcctttcccagagtttcccctggtttttaaaaaaagaaaattatgatactcaattggcttagtaaaatctcacatttagccagcttagctgaaacatttcagacctatgtttattatacaaggggtttttgtttgtttgtttgtttgtttgtttagggtgagatgaaagaggcaagatttaagaagctgggcaaaaactgagctgatgctggcctttaaagtacctcccaccttgctcaaccccagcaggagaggaataagaagagtttggaagggataatgataccatatgaagcaagagaggacagaaacaggagagtcgagaagcaggatctctagcagtatgcccttgaaggcagagactgcagtcagcgatcggcctaagctctgcacacacggcaatggcaatttgtccaatgagccctgttgaaggtggagtgctgctgcctgtacctcctcatcatcactgttgcttgagcaccgaagaagagtggcccagccttttgggtgcagctgtaaggacgtgatgcagtttccgtggtcactctcaccaagaacttcaggggttacgacttcaagactatttcgtggtgaaactcctgaacttgaagtagttcttcttgctcttaaaatgggatagctgcctacttctaaagacttagttaagtcaaggtcatgcaaaattaagagatatccagaggacgttgaaatcaacattttggaacaatctggtgttaacctcattcgcatgagaaaacgtgtgtgaaagaatttcttatgtggacacccatcttctgtatacctgttagtgtcccaaataatgacatttccatcaaatcctgatgttactaagagtcttgtattagtatcatattcgatgttcttcacccagctagtgtgaccatgtaaagtgcatactttggtgttcaattttctcagatcccatagtgctattgtagtgtcatcagagcaggtagcaaacagccggttatcaagaaatctgatattatttacacagtcttcatgagcttcagaaagtgtttttatgtgctttgaagatatagggtcaaaaagcagaacttcagtttgttcacaagcaactgtcagcactgacccgtcgggcgagtactcgaggttgaagacggcgccgtgggtgcgggtgctgaggtacaccgagtccgcggggtggatggaaccgtagaggctagtcatggtgcgaaaattgtcccgcgccgggtccacgaacagcccgcggcccaggctgcgctctttcagccacccgaacagcctagcgccagggccgcccaggcccgcgccgaggccgtgtcggccccggctcttggccctgcagtctggcccgggccgccggcacggaggggagggaggtgacggctctcccggggcggaggcagttgaggactccggagctccaggcagccctagctctccggagcgcggggccggggacagcgatggggcgccggggcggcgagggcttcgggcgggtggagggggatgggtcgcatcagccccgggatgtagtggcgagggcggcccggtggctgctgcctgcccctcgtggggcgtcggctcctcagccccggctccggccgatccgtcccctccagggctatggggcccaaagggaaacatgatcaacgcccccgccccccgctccgggccactgccccgccggccgacacctcagtgcccctgttcagctgccacttccggcgtgcagcggcctaaccccac

SEQ ID NO: 13735 - RNA, 5215 nt, Homo sapiens
  source 1..5215: mol_type = other RNA
gctgggattacaggcatgagccaccatgcccagtctatttttattttttgagacaggatctggctctattgcccagggtggagtgcaatagtgcaatcttggctcactgcagcctctgcctcccaggctcaaaccatcctcccacctcagcctcctgagtagctaggactacaggcgtgtaccaacatgcccatctaatttttgtatttttggtagagatggggtttcgccatgttgcccagactggtctggaactcctgggctcaagtgaacctcccaccttggcctcccaaagtgctgggattacagacgtgagccaccatacccatccctattttctttaaaaaatgtgttttttacaaaatgtatggtaagtatatgtatttactgtgctttgtgataattttctcagtgacaaaaaatttccaattttgttaacatccatggtaaaatgatctaatttcaaaaatttgttctagagccaagatccttataacctctataaatgtgtgtgaatagttagttggcaggtcctacaaagaaatgtcatttttattcatgtattttgggttgtttaaacatttctgtaagatttaaaatacttttcttcttatggctagaattctcagcatctactcccatgcctgcctttctaaaatctattggccagtttaagggtatttacaataatacaacttaaagacaaagtgtccataagtcattatttctaacagacagcataacacagtagaaattgccctgaccaaggaattagaagactggaattcaagtcctaactctgccactaactttgcaggatgaccttaggcaagtcatgtcacttctctcatttgtcaaataatgcaaatgattccattctaaggtattttccacctctaaaattgctttcatttactattattattttttaaataatgaaaacactttctgggaattgtcttaagcccaaatgggtagagaagaattttttttttttttttttttttttgagacagagtctcgctctgtcgcctaggctggagtgcagtggtgcaatctcggcttactgcaccctctgcctcccgggttcaagtgattctcttgcctcagcctcctgggtagctgggattacaggtgagcaccaccacgcccggctaatttttgtatttttagtagagatggcgtttcaccatgttggtcaggctggtctcgaactcctgaccttgtgatccacccacctcggcctcccaaagtgctgggattacaggcatgagccactgcgcctggccgagtagagaagaatttactgctgattaaggttgtgtttttcaacctgcaatcccgagaccctcagaataaagattacttgaggttgctatgaaaaatacagattcctgtcctccccctggctgaatcagaatctcataaggtgaggctcaggtttctgcacttttcacaagctctgtaatggttacagtgcaccctaatgtttgagaaccagtggcctaaagagaatgcaacctaagagggcaaggctagtgcatagcttaaatcgctccagcctttggtaatcccttctaaacacagtaccacccatgtggaggagactgcaaggaagctgttattcaaagtagaacagtcagccttgtgcttgagtcctgctttatgcttgcgtgtttcataacaaaacacaaaggcaagtcttcatatcagcacttagtcttgatatccaagtagctgactactgtacttatgataacagcttgaagaggactgcaactctcccctcacgaatggtgacagagttggcttgtcacacctggctcagggaagaaaaatgagtaaacccctacctctttactcttgattcctcttccaccctaatactgttaacacatcatcctgtgtgattcaaataatctggcagatgaaatacagaaaatctaagtcatattgttcttatcactctatggccagatattatactaatctaattttaaaaatccttttctgtgcaatagaaataaccaaagctcattctgtctcctttcctttctaatgctgttgataggaacaaaatatcaagtaaggatacatgctagagatgttaaattcatacaagtaaagtaaattacaaagagaggtggtaatatttttttctagaatttcacaataaaatccctctcaccatgaaaatctttttataattttaacaggaaacttaaaagacattttgttgcaagactatcttaacaattataagaataatgccattatctgtgctcaatatagataaacataacagtaactttaaaaggccaagtatactcataagtgaggatgaaatttatttttcaacaaccaatatgccaatatccaacttctaggttttattcaattctaatgtcatgggtttctcctaccccagtcaaaactcctgccaaatgtccacaaaattgacaccaaaatcaacaaacacaaagaaagagagggacagggagagggaaagagaaatagagagtgaggaaggaaggaacgtgacaagagctaccatgcaaaatgaccagaagaactggagttcagtggcacagatcagcaggagcagaggaatgctgcaaaagatgatgctgcatagagtctaacttggagatgcctgtatgatgctggatgaccaagtactaaggtcacaagtgtgttcatggacccataagaaccaggatcttgacccaaacttataagatcttctaaaaagaaaatacttcatctaaattgaagcaattcctaagtcaaacaccagaagagttccttatttgatgtaagttgtgcctaaaactttggctgatacaaagaaacccgtccactaaggcaccctgaggcaatctgacaatgtgttggagagaactttgttgtcagtaccacatcattatgagagtacagagaacggatcacccgcaggggactggcttctttgggcaagcagtcaacaagttcactgcactgtttgtcaaatcccaacaagcgaatcccatagccatgtggggaagaaatcattcgtccatcggggctgaagcaaagttctttgatgtaacccctgcctacattggcttcttcaatgtaatgagtcagtcgtagagaacagcgaggtgagacaggtcgcactggagctccttcttggaattcatagacacaagtacactcttcccctacacaattcaaaggctcttctcttctctcctttcagttgtggcctctaggaccagtgagatccttggaagactcttgctttccagagtgatgagaatcataaagtcatttaacacctttccccctagtcatcagtatagtcccttcctttcccagagtttcccctggtttttaaaaaaagaaaattatgatactcaattggcttagtaaaatctcacatttagccagcttagctgaaacatttcagacctatgtttattatacaaggggtttttgtttgtttgtttgtttgtttgtttagggtgagatgaaagaggcaagatttaagaagctgggcaaaaactgagctgatgctggcctttaaagtacctcccaccttgctcaaccccagcaggagaggaataagaagagtttggaagggataatgataccatatgaagcaagagaggacagaaacaggagagtcgagaagcaggatctctagcagtatgcccttgaaggcagagactgcagtcagcgatcggcctaagctctgcacacacggcaatggcaatttgtccaatgagccctgttgaaggtggagtgctgctgcctgtacctcctcatcatcactgttgcttgagcaccgaagaagagtggcccagccttttgggtgcagctgtaaggacgtgatgcagtttccgtggtcactctcaccaagaacttcaggggttacgacttcaagactatttcgtggtgaaactccttctctttgagaggctcgtgacatgtgtttctcagaagaattagaatcactatgatgacaaggtgagccagaaactctaggaccagatgaacttgatgaagtggtcaaatctgaacttgaagtagttcttcttgctcttaaaatgggatagctgcctacttctaaagacttagttaagtcaaggtcatgcaaaattaagagatatccagaggacgttgaaatcaacattttggaacaatctggtgttaacctcattcgcatgagaaaacgtgtgtgaaagaatttcttatgtggacacccatcttctgtatacctgttagtgtcccaaataatgacatttccatcaaatcctgatgttactaagagtcttgtattagtatcatattcgatgttcttcacccagctagtgtgaccatgtaaagtgcatactttggtgttcaattttctcagatcccatagtgctattgtagtgtcatcagagcaggtagcaaacagccggttatcaagaaatctgatattatttacacagtcttcatgagcttcagaaagtgtttttatgtgctttgaagatatagggtcaaaaagcagaacttcagtttgttcacaagcaactgtcagcactgacccgtcgggcgagtactcgaggttgaagacggcgccgtgggtgcgggtgctgaggtacaccgagtccgcggggtggatggaaccgtagaggctagtcatggtgcgaaaattgtcccgcgccgggtccacgaacagcccgcggcccaggctgcgctctttcagccacccgaacagcctagcgccagggccgcccaggcccgcgccgaggccgtgtcggccccggctcttggccctgcagtctggcccgggccgccggcacggaggggagggaggtgacggctctcccggggcggaggcagttgaggactccggagctccaggcagccctagctctccggagcgcggggccggggacagcgatggggcgccggggcggcgagggcttcgggcgggtggagggggatgggtcgcatcagccccgggatgtagtggcgagggcggcccggtggctgctgcctgcccctcgtggggcgtcggctcctcagccccggctccggccgatccgtcccctccagggctatggggcccaaagggaaacatgatcaacgcccccgccccccgctccgggccactgccccgccggccgacacctcagtgcccctgttcagctgccacttccggcgtgcagcggcctaaccccac

SEQ ID NO: 13736 - RNA, 7882 nt, Homo sapiens
  source 1..7882: mol_type = other RNA
gctgggattacaggcatgagccaccatgccccaccaagacaaacaaaacaaaacaaaacaaaacaaaacaaaacaaaaacagtatagatgaaaggcagccagcctgggttcaaatcctaccgttgctacttattattaaataaacgtaagaatcttatggacgttactttacctctctagcaccttgactttcaaatctgcaaaacaggataataacacctatttctttataacattgttataaggattaagtaggttaatatatgtgaaatacttagagtaatgtctggtacacagtaggcactaaataagtgttagcagccaggtgcggtggctcacaaggtcaggagtttgtgaccacactggccaacatagtgaaaccctgtctctactaaaaatataaaaattagctgggcatggtggcgtgtgcctgtagtcccagctactcgggaggctgaggcaggagaatcacttaaacccggaaggcggcggttgtggtgagctgagatcgcaccactgcactccagcccaagcaacagagcgagactccgtctcaaaaaaaaaaaaaaaaaaaaaagtatagctactattataatcctgtgaaaataatcaatataaaattaaaaatcaacagacagcccatattgcccttttttggcctaacaaaaaacagatttctaagaagacagtaagaaatcagtattaatttaaacattgtacaggacaggagatcaaaagcacaggtatacaaatggttcatttaaaaaaactgatactcaaattgacaccctgaaaatgtcagataatttttcagaatgattaaactcactaaacatctgtaaacaataaatttatttcatttcttttaaagatttaatgatatacaaaacgtatatagtatctttaagtaatacactttttctttctccccacccccaatcaatattaaacactatttaaacagcttatcatctcttgccttgtctgtatctatgagatacactactaaatacaaataagctttatactgctcccttccaaataaaaattaaaattagtaccaaggaaacaaaagaaaaagaaaaaaaaagaaaaaaaattaaagcataaaacttagatgaaaagcttttcttgttattgttgaatattcaacaatatctggggctgttaaattacattttattggcataaggttgcactgcaatctgccagtatcacataatgataatccaactgaattaatttcttaagtaccacaaacagcattcatgttcaaatgttccaacacaattttaaatatatgcaagagttcatgtttacattctgatttgatataacaatcaataaaatctttggagaagtttgtaagttctgggttgttgctatagatacagatagggaaaaaagtactttaactttcctcaaaaggtaacttcccttgacgagtgagttaggtttctgcttttataatttaggttatgtatcagtttaccatggctttcttctacttaacagtgacttgataaaacaatgtttaaaaaacccaattaacatttttacacaatttgggttctatttaaaaaaaaaaactggctctatctttaaatatggagcctaaccctgattcataaataccgtccctcttgaaaatggtcttcagttcaggcttctcatacctctgtgaacctagaattagaacaagtcatttcccttcccgtggccaacaagcatctagttgggaaccagtgatatcatcactgaacacactaaatacactgaggaaaattttgactgccatttaaccaaaaggctgcgtgatttcttcatttccctagttgaatggcaataaaacagctgccaataaaatctgcatggacacctacctttggttaatggtattgtaccacataagagagagcatcaccctcatcaaaacaaagtcaaatgagatcctctgctatacaaagagccctttaaaaagttataaatactaattatcaattacctttaaaatttctcagctgccagctctatcctatagggactttctgactgattaatcaggtcaaaagaatattgaccttttaactgtgctggagtcagcaaattcaacttgcatacacctttctatattaccaaacaatttcctcccgagggaaaagtgacacagtaacatttctgtgaggtgcaggcaaaaccaatgattcagtaatattaatattataacatcagacgaacagaattagttgattctgattctttggtggaatttccaggctgaagattcaaatctgaaggctcatcctgaggaaatataattttatcaggcgtataatcattcctcttcagatctggaagtttaagctttctacagcaagaattacagtgatgttttgctctgaagtttttaattgcatcttctcctagatttgctgggccaaaaaccatatcacaggatctcttttcttctgcttttatcacagatgggtcagtcaaattttcaccaacaccttgcaaatcaagtaccagtaactcccctcttgtatattcgtaagtccagtggctaaaggctagcatgatctcttccagagtattagttggaataatctcatctccattattattgttgtattttctaaattctccagtcatacattcttccacagcaaaccactgtcctgctgaatggcaatacagcaggaaaacttcaaggaaccttggagaatatggtatggatttgggtttcatttgattaaaggcaaacgtaagcttttgtgctgctctctgttgttgaatttctctcagacagagatgcagaactgtatcttctttgtaaatacttgaccatgtattaaccacctctggaagaaaagatttgataatataaagatgccctgatttgaggatatcatgttctgaccaggtacactgtactttgacagctcttcgtaaacctcctcccatctcctctttgcttaaaaactctattttggcacagaggcctagttgtgaccaagaagacatgctgttatttagtatgttgggtgaactctcttccaaacgatacactgtgacaggctcccctcttggaggcacaggtgtaaatggaatgctctgtgataacctcatcaagttatttctttccacagctgaataatagtaatttgtatccatagctggcttaaatggagaagtgagaccatttaatgttccttcttcagatggcatttctctgtttgatggtctatcttgtaaccaatccggtattaaagctgctttggaatctacttcatgagtgtcttcggtagatggccttctactgattttttctgcttgttttgaatgaacaggaatggaagttctgtgacagtcagtaaatccagcaagagaactcactcgtttcaaagtgttttcagaagtattgttattggatagtatttttatcttgtttgatgtttctttaaacctctgtaaatccatgctatctctgtgtcctacaaatgctccaaattctgtattatctccttctgtagctttagagcaaacagtttcttgatctttggttccagtttccaagtggcttttgcaacttggctgagatggtgtactaacaaaaaatttggttggtggggatgacagatgtggtatgctagtagatgaactgcctaatttttgatttttattaaatatttttaagagttctaccccatgtagtctctgtcgcagttctggaggggaaacagcacttgggaataaggcaccagaagaggaaccagcctctggaaaattaaattcttttctctggggtactgcaggtaagtcttgaccaaatatattacactggggatctttgtcatctttcattaaaatattacaatgaaaaggattattactttcaagatcaccttgaggaagagaggagctaagtgtatttacaacaccatgctttttccatacagaaggtcttacaggaccatcatcaataaggttttgagccaagtgtttggaaatgctcagttctcgtgtgatttcattatgaactttgctagcttccgacgctttctgggcagtgagtgtttttaatgtatctaccgtcagggctgaaagatcttgcaaatggccaatttgagaatctaatgattgtaatgatctttttatgtagttgacacgatctccaacttctttaatctgaatgcacatctgttccactctttcaaaagtgacacgaattctctcttcactcccagaatgaaatttgtcatctttttcattgaaatacatttcaacacactgctcttcaaaatcatgaagtttcttttgatcttcttctgttaagaaaagttttggtccatcggaagtcttatctttctttcttctcttacatatgcagcaaaacagagaaactatatggctaagaatgataagtggaggaggcagaactggtttctcatgataagccataataaaatgataacgctggtacttccatacaatattggaaattgccttcacttgtaaatacacattgcatcaatttcgtatgcataaacttcaccaaaaatcatccagtatgggtgaaaaactatatctttagcaagagtccaagatggtgcttcatgaggataaagtattgcctttctgggaacaccaaaactaagtaatacaagagccataatcactacaatgtagaacatattggccaccaaaatattatgttaagacagtaaattaatcttccagccacaaaaacatgattatcatatgcatttgcaaagttccattttgctccaaatcttagtccaaatccaatgaagaaagaaattatggcaattgtatcactgatgttgaagtaatcactaaaccatactttaatcttctggtttactttcccagcttcagacataaagatctcacggactttctcaatggcataagtaaaaatataagcaataacaatccattcttgaactgaaggtaactgttccatttgtacaagaaccacaaatgtataaagcatcagaaatcctaaatatgccaacgtgttaaaccagaattttacaattggtgcatgataaaaggcataaaactttcgcgtaattggaagcttttttgatttcatttgtatctccatctcattctttccttcattactatccaaaatccgtacttctttaaacacttccatggggatctcttctgttatgttctgaaagttgttttcgctgtcatccattgtcatctgatgagcatcttgagattgtgggatatgggacatttcagccttagttttatactctaacagcaatatggcaggtggaactaaaatgcttagtatgaccttgtaccaggaatttttcctcatattcagccttcccatccacatatcagataacaacatttgtgtacaggtgtgagctacaaaaggtctaagtcttgaagaaactgctaacttaaggcaggttgaattactccagttcttcagttcataagtgagcaatttcatagccatggtttcatcttgtctgaaggactgttctaataattcaacggccaactgaccaaaatcattggaatactgttttagttcttctgaagtatcatctaccaggtcactctgctttgcttcatatgccattgaacgatagatcttacaggcaactaatgctttagccattgattcttcaccatgttgccataaaaaacgggccatgacctgcctcttcataaggcaagcccaaattaaaagttcattaagtggataaggaaagcgcttggtttctggatcatcaatgtctacaatttcatctttggttcttttcttctttccttcttccataactgtatcaatctttggtcggtagggctgtgctgtcttaatgaaatggttatgcctcattttttcctttttatctgccctattgccaaaagattcatgactctttcgcaactgaggagtgctgctggaggtatttcggccagacctccgattatttccaccaagactattatatattaatcgaaaacgtttcctagtataggtgcatctgtaggttcctcccatgagatattcaataacaagtcctatatcaatcagagtgatcttatatcctggaggaagatttccctgtttgacgtctcgaacaagatgaaacagcattggattagttggaccttgtttagtgttgtaaagttcttccagtctcggaatggtaaggaatttatgcatgcttactccattttcaataagaagttttacaaatgcaactctatccattacaagagcatcaagcatagcttgttccaaggatccaaccagccactgctgtccataaacaaatacatgatttttggcaatgtcaactctatcccatgccaatgtaaggataagctggtcaaatgcagatgcattagtaccttttagcagtgcagtaagtattgctacatctatatcttgatgttcatctgacccaatatggaaaacagtgataagctcctttcttttcatgcactccatcagtgtttgaaataaatgaagtgcttcattctggccaaagttaaatgtttttttgatagtggaaataatatcgggctctgctgcatcaggaagattccctccttcttctgtttgtttatgaatatacgctagcagatctgcagctctgcctgttccttcacacacaactactggaacaggggggctttcctgaaggtattcaagaactgtgaggataacatttggcccaccctcaaatataagtgccaccacagggacaccctggccaatcctagcatgaattctttgctgattaatagttttttcaagttctcttctcagtctgacttccgccccatactttccaacagtgccatcatccaccaatatgaaatgggaatgcagattattcaaaacattcaatttgctcagggggttcaataaggtttgataaggagcaaccacatctctcccaacaagatcatttctgttttcaatcactccccatggagctattccgatagtgcaaatctttcgagatgatctggaagcatgttctttgagggcatctccaacatgttttgccacacctgtgtttactcctccagttaaaatccaggctccagttgtaactgcagctttaataagaccttttccaagcaactgcttgattcgtgggtgaagctcaaatttctgcatgcccccatgtacagagataacaagtttgggtaactccatttgccattctttaagcagaagttgcagaatgacttcaggtttggtgtcatatgatagcctcacatacttagctctgtaggaatgagaacccccttgaaaatttatgactccataagcatccgttgggctctgttctgtatgcttttccacagaccattcttctattgcctgattaaaatggtcacccaatttcacatctgagtatttcatggcaagacttgcagtaaaacaagcatgttgcttgaccaagcgaccacaaaaacacctgacgagttgctgacaaatttgacatcctggaaggcatctgtgagggtccttggaacttggtataatatatacacattccctcttggtcaaagtgctttctatccaggatttctgggacattctcctcacggggcggactccggaagggcagcaactccacctcctcctcctccgcggcctgtagccatctatcgggaagcgtctccggaggcggcagcagaggccgccggacaaggaacgcccagggaaaccttctcagaactaactcagctccggcgctagcagcagaagccgagtctttcataattgtgcgaccaactcctccgggtgactggccacagggacgcgcccgcgcccgcctccgccggcgacggggctggggac

SEQ ID NO: 13737 - RNA, 7955 nt, Homo sapiens
  source 1..7955: mol_type = other RNA
gctgggattacaggcatgagccaccatgccccaccaagacaaacaaaacaaaacaaaacaaaacaaaacaaaacaaaaacagtatagatgaaaggcagccagcctgggttcaaatcctaccgttgctacttattattaaataaacgtaagaatcttatggacgttactttacctctctagcaccttgactttcaaatctgcaaaacaggataataacacctatttctttataacattgttataaggattaagtaggttaatatatgtgaaatacttagagtaatgtctggtacacagtaggcactaaataagtgttagcagccaggtgcggtggctcacaaggtcaggagtttgtgaccacactggccaacatagtgaaaccctgtctctactaaaaatataaaaattagctgggcatggtggcgtgtgcctgtagtcccagctactcgggaggctgaggcaggagaatcacttaaacccggaaggcggcggttgtggtgagctgagatcgcaccactgcactccagcccaagcaacagagcgagactccgtctcaaaaaaaaaaaaaaaaaaaaaagtatagctactattataatcctgtgaaaataatcaatataaaattaaaaatcaacagacagcccatattgcccttttttggcctaacaaaaaacagatttctaagaagacagtaagaaatcagtattaatttaaacattgtacaggacaggagatcaaaagcacaggtatacaaatggttcatttaaaaaaactgatactcaaattgacaccctgaaaatgtcagataatttttcagaatgattaaactcactaaacatctgtaaacaataaatttatttcatttcttttaaagatttaatgatatacaaaacgtatatagtatctttaagtaatacactttttctttctccccacccccaatcaatattaaacactatttaaacagcttatcatctcttgccttgtctgtatctatgagatacactactaaatacaaataagctttatactgctcccttccaaataaaaattaaaattagtaccaaggaaacaaaagaaaaagaaaaaaaaagaaaaaaaattaaagcataaaacttagatgaaaagcttttcttgttattgttgaatattcaacaatatctggggctgttaaattacattttattggcataaggttgcactgcaatctgccagtatcacataatgataatccaactgaattaatttcttaagtaccacaaacagcattcatgttcaaatgttccaacacaattttaaatatatgcaagagttcatgtttacattctgatttgatataacaatcaataaaatctttggagaagtttgtaagttctgggttgttgctatagatacagatagggaaaaaagtactttaactttcctcaaaaggtaacttcccttgacgagtgagttaggtttctgcttttataatttaggttatgtatcagtttaccatggctttcttctacttaacagtgacttgataaaacaatgtttaaaaaacccaattaacatttttacacaatttgggttctatttaaaaaaaaaaactggctctatctttaaatatggagcctaaccctgattcataaataccgtccctcttgaaaatggtcttcagttcaggcttctcatacctctgtgaacctagaattagaacaagtcatttcccttcccgtggccaacaagcatctagttgggaaccagtgatatcatcactgaacacactaaatacactgaggaaaattttgactgccatttaaccaaaaggctgcgtgatttcttcatttccctagttgaatggcaataaaacagctgccaataaaatctgcatggacacctacctttggttaatggtattgtaccacataagagagagcatcaccctcatcaaaacaaagtcaaatgagatcctctgctatacaaagagccctttaaaaagttataaatactaattatcaattacctttaaaatttctcagctgccagctctatcctatagggactttctgactgattaatcaggtcaaaagaatattgaccttttaactgtgctggagtcagcaaattcaacttgcatacacctttctatattaccaaacaatttcctcccgagggaaaagtgacacagtaacatttctgtgaggtgcaggcaaaaccaatgattcagtaatattaatattataacatcagacgaacagaattagttgattctgattctttggtggaatttccaggctgaagattcaaatctgaaggctcatcctgaggaaatataattttatcaggcgtataatcattcctcttcagatctggaagtttaagctttctacagcaagaattacagtgatgttttgctctgaagtttttaattgcatcttctcctagatttgctgggccaaaaaccatatcacaggatctcttttcttctgcttttatcacagatgggtcagtcaaattttcaccaacaccttgcaaatcaagtaccagtaactcccctcttgtatattcgtaagtccagtggctaaaggctagcatgatctcttccagagtattagttggaataatctcatctccattattattgttgtattttctaaattctccagtcatacattcttccacagcaaaccactgtcctgctgaatggcaatacagcaggaaaacttcaaggaaccttggagaatatggtatggatttgggtttcatttgattaaaggcaaacgtaagcttttgtgctgctctctgttgttgaatttctctcagacagagatgcagaactgtatcttctttgtaaatacttgaccatgtattaaccacctctggaagaaaagatttgataatataaagatgccctgatttgaggatatcatgttctgaccaggtacactgtactttgacagctcttcgtaaacctcctcccatctcctctttgcttaaaaactctattttggcacagaggcctagttgtgaccaagaagacatgctgttatttagtatgttgggtgaactctcttccaaacgatacactgtgacaggctcccctcttggaggcacaggtgtaaatggaatgctctgtgataacctcatcaagttatttctttccacagctgaataatagtaatttgtatccatagctggcttaaatggagaagtgagaccatttaatgttccttcttcagatggcatttctctgtttgatggtctatcttgtaaccaatccggtattaaagctgctttggaatctacttcatgagtgtcttcggtagatggccttctactgattttttctgcttgttttgaatgaacaggaatggaagttctgtgacagtcagtaaatccagcaagagaactcactcgtttcaaagtgttttcagaagtattgttattggatagtatttttatcttgtttgatgtttctttaaacctctgtaaatccatgctatctctgtgtcctacaaatgctccaaattctgtattatctccttctgtagctttagagcaaacagtttcttgatctttggttccagtttccaagtggcttttgcaacttggctgagatggtgtactaacaaaaaatttggttggtggggatgacagatgtggtatgctagtagatgaactgcctaatttttgatttttattaaatatttttaagagttctaccccatgtagtctctgtcgcagttctggaggggaaacagcacttgggaataaggcaccagaagaggaaccagcctctggaaaattaaattcttttctctggggtactgcaggtaagtcttgaccaaatatattacactggggatctttgtcatctttcattaaaatattacaatgaaaaggattattactttcaagatcaccttgaggaagagaggagctaagtgtatttacaacaccatgctttttccatacagaaggtcttacaggaccatcatcaataaggttttgagccaagtgtttggaaatgctcagttctcgtgtgatttcattatgaactttgctagcttccgacgctttctgggcagtgagtgtttttaatgtatctaccgtcagggctgaaagatcttgcaaatggccaatttgagaatctaatgattgtaatgatctttttatgtagttgacacgatctccaacttctttaatctgaatgcacatctgttccactctttcaaaagtgacacgaattctctcttcactcccagaatgaaatttgtcatctttttcattgaaatacatttcaacacactgctcttcaaaatcatgaagtttcttttgatcttcttctgttaagaaaagttttggtccatcggaagtcttatctttctttcttctcttacatatgcagcaaaacagagaaactatatggctaagaatgataagtggaggaggcagaactggtttctcatgataagccataataaaatgataacgctggtacttccatacaatattggaaattgccttcacttgtaaatacacattgcatcaatttcgtatgcataaacttcaccaaaaatcatccagtatgggtgaaaaactatatctttagcaagagtccaagatggtgcttcatgaggataaagtattgcctttctgggaacaccaaaactaagtaatacaagagccataatcactacaatgtagaacatattggccaccatttttccaatcatcattacataaggtcctgcctgttgatttacagctagaaaatctagcaaacgcacataccaaaatattatgttaagacagtaaattaatcttccagccacaaaaacatgattatcatatgcatttgcaaagttccattttgctccaaatcttagtccaaatccaatgaagaaagaaattatggcaattgtatcactgatgttgaagtaatcactaaaccatactttaatcttctggtttactttcccagcttcagacataaagatctcacggactttctcaatggcataagtaaaaatataagcaataacaatccattcttgaactgaaggtaactgttccatttgtacaagaaccacaaatgtataaagcatcagaaatcctaaatatgccaacgtgttaaaccagaattttacaattggtgcatgataaaaggcataaaactttcgcgtaattggaagcttttttgatttcatttgtatctccatctcattctttccttcattactatccaaaatccgtacttctttaaacacttccatggggatctcttctgttatgttctgaaagttgttttcgctgtcatccattgtcatctgatgagcatcttgagattgtgggatatgggacatttcagccttagttttatactctaacagcaatatggcaggtggaactaaaatgcttagtatgaccttgtaccaggaatttttcctcatattcagccttcccatccacatatcagataacaacatttgtgtacaggtgtgagctacaaaaggtctaagtcttgaagaaactgctaacttaaggcaggttgaattactccagttcttcagttcataagtgagcaatttcatagccatggtttcatcttgtctgaaggactgttctaataattcaacggccaactgaccaaaatcattggaatactgttttagttcttctgaagtatcatctaccaggtcactctgctttgcttcatatgccattgaacgatagatcttacaggcaactaatgctttagccattgattcttcaccatgttgccataaaaaacgggccatgacctgcctcttcataaggcaagcccaaattaaaagttcattaagtggataaggaaagcgcttggtttctggatcatcaatgtctacaatttcatctttggttcttttcttctttccttcttccataactgtatcaatctttggtcggtagggctgtgctgtcttaatgaaatggttatgcctcattttttcctttttatctgccctattgccaaaagattcatgactctttcgcaactgaggagtgctgctggaggtatttcggccagacctccgattatttccaccaagactattatatattaatcgaaaacgtttcctagtataggtgcatctgtaggttcctcccatgagatattcaataacaagtcctatatcaatcagagtgatcttatatcctggaggaagatttccctgtttgacgtctcgaacaagatgaaacagcattggattagttggaccttgtttagtgttgtaaagttcttccagtctcggaatggtaaggaatttatgcatgcttactccattttcaataagaagttttacaaatgcaactctatccattacaagagcatcaagcatagcttgttccaaggatccaaccagccactgctgtccataaacaaatacatgatttttggcaatgtcaactctatcccatgccaatgtaaggataagctggtcaaatgcagatgcattagtaccttttagcagtgcagtaagtattgctacatctatatcttgatgttcatctgacccaatatggaaaacagtgataagctcctttcttttcatgcactccatcagtgtttgaaataaatgaagtgcttcattctggccaaagttaaatgtttttttgatagtggaaataatatcgggctctgctgcatcaggaagattccctccttcttctgtttgtttatgaatatacgctagcagatctgcagctctgcctgttccttcacacacaactactggaacaggggggctttcctgaaggtattcaagaactgtgaggataacatttggcccaccctcaaatataagtgccaccacagggacaccctggccaatcctagcatgaattctttgctgattaatagttttttcaagttctcttctcagtctgacttccgccccatactttccaacagtgccatcatccaccaatatgaaatgggaatgcagattattcaaaacattcaatttgctcagggggttcaataaggtttgataaggagcaaccacatctctcccaacaagatcatttctgttttcaatcactccccatggagctattccgatagtgcaaatctttcgagatgatctggaagcatgttctttgagggcatctccaacatgttttgccacacctgtgtttactcctccagttaaaatccaggctccagttgtaactgcagctttaataagaccttttccaagcaactgcttgattcgtgggtgaagctcaaatttctgcatgcccccatgtacagagataacaagtttgggtaactccatttgccattctttaagcagaagttgcagaatgacttcaggtttggtgtcatatgatagcctcacatacttagctctgtaggaatgagaacccccttgaaaatttatgactccataagcatccgttgggctctgttctgtatgcttttccacagaccattcttctattgcctgattaaaatggtcacccaatttcacatctgagtatttcatggcaagacttgcagtaaaacaagcatgttgcttgaccaagcgaccacaaaaacacctgacgagttgctgacaaatttgacatcctggaaggcatctgtgagggtccttggaacttggtataatatatacacattccctcttggtcaaagtgctttctatccaggatttctgggacattctcctcacggggcggactccggaagggcagcaactccacctcctcctcctccgcggcctgtagccatctatcgggaagcgtctccggaggcggcagcagaggccgccggacaaggaacgcccagggaaaccttctcagaactaactcagctccggcgctagcagcagaagccgagtctttcataattgtgcgaccaactcctccgggtgactggccacagggacgcgcccgcgcccgcctccgccggcgacggggctggggac

SEQ ID NO: 13738 - RNA, 8032 nt, Homo sapiens
  source 1..8032: mol_type = other RNA
gctgggattacaggcatgagccaccatgccccaccaagacaaacaaaacaaaacaaaacaaaacaaaacaaaacaaaaacagtatagatgaaaggcagccagcctgggttcaaatcctaccgttgctacttattattaaataaacgtaagaatcttatggacgttactttacctctctagcaccttgactttcaaatctgcaaaacaggataataacacctatttctttataacattgttataaggattaagtaggttaatatatgtgaaatacttagagtaatgtctggtacacagtaggcactaaataagtgttagcagccaggtgcggtggctcacaaggtcaggagtttgtgaccacactggccaacatagtgaaaccctgtctctactaaaaatataaaaattagctgggcatggtggcgtgtgcctgtagtcccagctactcgggaggctgaggcaggagaatcacttaaacccggaaggcggcggttgtggtgagctgagatcgcaccactgcactccagcccaagcaacagagcgagactccgtctcaaaaaaaaaaaaaaaaaaaaaagtatagctactattataatcctgtgaaaataatcaatataaaattaaaaatcaacagacagcccatattgcccttttttggcctaacaaaaaacagatttctaagaagacagtaagaaatcagtattaatttaaacattgtacaggacaggagatcaaaagcacaggtatacaaatggttcatttaaaaaaactgatactcaaattgacaccctgaaaatgtcagataatttttcagaatgattaaactcactaaacatctgtaaacaataaatttatttcatttcttttaaagatttaatgatatacaaaacgtatatagtatctttaagtaatacactttttctttctccccacccccaatcaatattaaacactatttaaacagcttatcatctcttgccttgtctgtatctatgagatacactactaaatacaaataagctttatactgctcccttccaaataaaaattaaaattagtaccaaggaaacaaaagaaaaagaaaaaaaaagaaaaaaaattaaagcataaaacttagatgaaaagcttttcttgttattgttgaatattcaacaatatctggggctgttaaattacattttattggcataaggttgcactgcaatctgccagtatcacataatgataatccaactgaattaatttcttaagtaccacaaacagcattcatgttcaaatgttccaacacaattttaaatatatgcaagagttcatgtttacattctgatttgatataacaatcaataaaatctttggagaagtttgtaagttctgggttgttgctatagatacagatagggaaaaaagtactttaactttcctcaaaaggtaacttcccttgacgagtgagttaggtttctgcttttataatttaggttatgtatcagtttaccatggctttcttctacttaacagtgacttgataaaacaatgtttaaaaaacccaattaacatttttacacaatttgggttctatttaaaaaaaaaaactggctctatctttaaatatggagcctaaccctgattcataaataccgtccctcttgaaaatggtcttcagttcaggcttctcatacctctgtgaacctagaattagaacaagtcatttcccttcccgtggccaacaagcatctagttgggaaccagtgatatcatcactgaacacactaaatacactgaggaaaattttgactgccatttaaccaaaaggctgcgtgatttcttcatttccctagttgaatggcaataaaacagctgccaataaaatctgcatggacacctacctttggttaatggtattgtaccacataagagagagcatcaccctcatcaaaacaaagtcaaatgagatcctctgctatacaaagagccctttaaaaagttataaatactaattatcaattacctttaaaatttctcagctgccagctctatcctatagggactttctgactgattaatcaggtcaaaagaatattgaccttttaactgtgctggagtcagcaaattcaacttgcatacacctttctatattaccaaacaatttcctcccgagggaaaagtgacacagtaacatttctgtgaggtgcaggcaaaaccaatgattcagtaatattaatattataacatcagacgaacagaattagttgattctgattctttggtggaatttccaggctgaagattcaaatctgaaggctcatcctgaggaaatataattttatcaggcgtataatcattcctcttcagatctggaagtttaagctttctacagcaagaattacagtgatgttttgctctgaagtttttaattgcatcttctcctagatttgctgggccaaaaaccatatcacaggatctcttttcttctgcttttatcacagatgggtcagtcaaattttcaccaacaccttgcaaatcaagtaccagtaactcccctcttgtatattcgtaagtccagtggctaaaggctagcatgatctcttccagagtattagttggaataatctcatctccattattattgttgtattttctaaattctccagtcatacattcttccacagcaaaccactgtcctgctgaatggcaatacagcaggaaaacttcaaggaaccttggagaatatggtatggatttgggtttcatttgattaaaggcaaacgtaagcttttgtgctgctctctgttgttgaatttctctcagacagagatgcagaactgtatcttctttgtaaatacttgaccatgtattaaccacctctggaagaaaagatttgataatataaagatgccctgatttgaggatatcatgttctgaccaggtacactgtactttgacagctcttcgtaaacctcctcccatctcctctttgcttaaaaactctattttggcacagaggcctagttgtgaccaagaagacatgctgttatttagtatgttgggtgaactctcttccaaacgatacactgtgacaggctcccctcttggaggcacaggtgtaaatggaatgctctgtgataacctcatcaagttatttctttccacagctgaataatagtaatttgtatccatagctggcttaaatggagaagtgagaccatttaatgttccttcttcagatggcatttctctgtttgatggtctatcttgtaaccaatccggtattaaagctgctttggaatctacttcatgagtgtcttcggtagatggccttctactgattttttctgcttgttttgaatgaacaggaatggaagttctgtgacagtcagtaaatccagcaagagaactcactcgtttcaaagtgttttcagaagtattgttattggatagtatttttatcttgtttgatgtttctttaaacctctgtaaatccatgctatctctgtgtcctacaaatgctccaaattctgtattatctccttctgtagctttagagcaaacagtttcttgatctttggttccagtttccaagtggcttttgcaacttggctgagatggtgtactaacaaaaaatttggttggtggggatgacagatgtggtatgctagtagatgaactgcctaatttttgatttttattaaatatttttaagagttctaccccatgtagtctctgtcgcagttctggaggggaaacagcacttgggaataaggcaccagaagaggaaccagcctctggaaaattaaattcttttctctggggtactgcaggtaagtcttgaccaaatatattacactggggatctttgtcatctttcattaaaatattacaatgaaaaggattattactttcaagatcaccttgaggaagagaggagctaagtgtatttacaacaccatgctttttccatacagaaggtcttacaggaccatcatcaataaggttttgagccaagtgtttggaaatgctcagttctcgtgtgatttcattatgaactttgctagcttccgacgctttctgggcagtgagtgtttttaatgtatctaccgtcagggctgaaagatcttgcaaatggccaatttgagaatctaatgattgtaatgatctttttatgtagttgacacgatctccaacttctttaatctgaatgcacatctgttccactctttcaaaagtgacacgaattctctcttcactcccagaatgaaatttgtcatctttttcattgaaatacatttcaacacactgctcttcaaaatcatgaagtttcttttgatcttcttctgttaagaaaagttttggtccatcggaagtcttatctttctttcttctcttacatatgcagcaaaacagagaaactatatggctaagaatgataagtggaggaggcagaactggtttctcatgataagccataataaaatgataacgctggtacttccatacaatattggaaattgccttcacttgtaaatacacattgttgaaaaatgcaataagaagattaaccataatgatatactgtacaaagaggtagactgcttgaagaaatggagtcaaccacgtcccaggaccacagatttgagggataacagaatcatttgcacacacatcaatttcgtatgcataaacttcaccaaaaatcatccagtatgggtgaaaaactatatctttagcaagagtccaagatggtgcttcatgaggataaagtattgcctttctgggaacaccaaaacatttttccaatcatcattacataaggtcctgcctgttgatttacagctagaaaatctagcaaacgcacataccaaaatattatgttaagacagtaaattaatcttccagccacaaaaacatgattatcatatgcatttgcaaagttccattttgctccaaatcttagtccaaatccaatgaagaaagaaattatggcaattgtatcactgatgttgaagtaatcactaaaccatactttaatcttctggtttactttcccagcttcagacataaagatctcacggactttctcaatggcataagtaaaaatataagcaataacaatccattcttgaactgaaggtaactgttccatttgtacaagaaccacaaatgtataaagcatcagaaatcctaaatatgccaacgtgttaaaccagaattttacaattggtgcatgataaaaggcataaaactttcgcgtaattggaagcttttttgatttcatttgtatctccatctcattctttccttcattactatccaaaatccgtacttctttaaacacttccatggggatctcttctgttatgttctgaaagttgttttcgctgtcatccattgtcatctgatgagcatcttgagattgtgggatatgggacatttcagccttagttttatactctaacagcaatatggcaggtggaactaaaatgcttagtatgaccttgtaccaggaatttttcctcatattcagccttcccatccacatatcagataacaacatttgtgtacaggtgtgagctacaaaaggtctaagtcttgaagaaactgctaacttaaggcaggttgaattactccagttcttcagttcataagtgagcaatttcatagccatggtttcatcttgtctgaaggactgttctaataattcaacggccaactgaccaaaatcattggaatactgttttagttcttctgaagtatcatctaccaggtcactctgctttgcttcatatgccattgaacgatagatcttacaggcaactaatgctttagccattgattcttcaccatgttgccataaaaaacgggccatgacctgcctcttcataaggcaagcccaaattaaaagttcattaagtggataaggaaagcgcttggtttctggatcatcaatgtctacaatttcatctttggttcttttcttctttccttcttccataactgtatcaatctttggtcggtagggctgtgctgtcttaatgaaatggttatgcctcattttttcctttttatctgccctattgccaaaagattcatgactctttcgcaactgaggagtgctgctggaggtatttcggccagacctccgattatttccaccaagactattatatattaatcgaaaacgtttcctagtataggtgcatctgtaggttcctcccatgagatattcaataacaagtcctatatcaatcagagtgatcttatatcctggaggaagatttccctgtttgacgtctcgaacaagatgaaacagcattggattagttggaccttgtttagtgttgtaaagttcttccagtctcggaatggtaaggaatttatgcatgcttactccattttcaataagaagttttacaaatgcaactctatccattacaagagcatcaagcatagcttgttccaaggatccaaccagccactgctgtccataaacaaatacatgatttttggcaatgtcaactctatcccatgccaatgtaaggataagctggtcaaatgcagatgcattagtaccttttagcagtgcagtaagtattgctacatctatatcttgatgttcatctgacccaatatggaaaacagtgataagctcctttcttttcatgcactccatcagtgtttgaaataaatgaagtgcttcattctggccaaagttaaatgtttttttgatagtggaaataatatcgggctctgctgcatcaggaagattccctccttcttctgtttgtttatgaatatacgctagcagatctgcagctctgcctgttccttcacacacaactactggaacaggggggctttcctgaaggtattcaagaactgtgaggataacatttggcccaccctcaaatataagtgccaccacagggacaccctggccaatcctagcatgaattctttgctgattaatagttttttcaagttctcttctcagtctgacttccgccccatactttccaacagtgccatcatccaccaatatgaaatgggaatgcagattattcaaaacattcaatttgctcagggggttcaataaggtttgataaggagcaaccacatctctcccaacaagatcatttctgttttcaatcactccccatggagctattccgatagtgcaaatctttcgagatgatctggaagcatgttctttgagggcatctccaacatgttttgccacacctgtgtttactcctccagttaaaatccaggctccagttgtaactgcagctttaataagaccttttccaagcaactgcttgattcgtgggtgaagctcaaatttctgcatgcccccatgtacagagataacaagtttgggtaactccatttgccattctttaagcagaagttgcagaatgacttcaggtttggtgtcatatgatagcctcacatacttagctctgtaggaatgagaacccccttgaaaatttatgactccataagcatccgttgggctctgttctgtatgcttttccacagaccattcttctattgcctgattaaaatggtcacccaatttcacatctgagtatttcatggcaagacttgcagtaaaacaagcatgttgcttgaccaagcgaccacaaaaacacctgacgagttgctgacaaatttgacatcctggaaggcatctgtgagggtccttggaacttggtataatatatacacattccctcttggtcaaagtgctttctatccaggatttctgggacattctcctcacggggcggactccggaagggcagcaactccacctcctcctcctccgcggcctgtagccatctatcgggaagcgtctccggaggcggcagcagaggccgccggacaaggaacgcccagggaaaccttctcagaactaactcagctccggcgctagcagcagaagccgagtctttcataattgtgcgaccaactcctccgggtgactggccacagggacgcgcccgcgcccgcctccgccggcgacggggctggggac

SEQ ID NO: 13739 - RNA, 8082 nt, Homo sapiens
  source 1..8082: mol_type = other RNA
gctgggattacaggcatgagccaccatgccccaccaagacaaacaaaacaaaacaaaacaaaacaaaacaaaacaaaaacagtatagatgaaaggcagccagcctgggttcaaatcctaccgttgctacttattattaaataaacgtaagaatcttatggacgttactttacctctctagcaccttgactttcaaatctgcaaaacaggataataacacctatttctttataacattgttataaggattaagtaggttaatatatgtgaaatacttagagtaatgtctggtacacagtaggcactaaataagtgttagcagccaggtgcggtggctcacaaggtcaggagtttgtgaccacactggccaacatagtgaaaccctgtctctactaaaaatataaaaattagctgggcatggtggcgtgtgcctgtagtcccagctactcgggaggctgaggcaggagaatcacttaaacccggaaggcggcggttgtggtgagctgagatcgcaccactgcactccagcccaagcaacagagcgagactccgtctcaaaaaaaaaaaaaaaaaaaaaagtatagctactattataatcctgtgaaaataatcaatataaaattaaaaatcaacagacagcccatattgcccttttttggcctaacaaaaaacagatttctaagaagacagtaagaaatcagtattaatttaaacattgtacaggacaggagatcaaaagcacaggtatacaaatggttcatttaaaaaaactgatactcaaattgacaccctgaaaatgtcagataatttttcagaatgattaaactcactaaacatctgtaaacaataaatttatttcatttcttttaaagatttaatgatatacaaaacgtatatagtatctttaagtaatacactttttctttctccccacccccaatcaatattaaacactatttaaacagcttatcatctcttgccttgtctgtatctatgagatacactactaaatacaaataagctttatactgctcccttccaaataaaaattaaaattagtaccaaggaaacaaaagaaaaagaaaaaaaaagaaaaaaaattaaagcataaaacttagatgaaaagcttttcttgttattgttgaatattcaacaatatctggggctgttaaattacattttattggcataaggttgcactgcaatctgccagtatcacataatgataatccaactgaattaatttcttaagtaccacaaacagcattcatgttcaaatgttccaacacaattttaaatatatgcaagagttcatgtttacattctgatttgatataacaatcaataaaatctttggagaagtttgtaagttctgggttgttgctatagatacagatagggaaaaaagtactttaactttcctcaaaaggtaacttcccttgacgagtgagttaggtttctgcttttataatttaggttatgtatcagtttaccatggctttcttctacttaacagtgacttgataaaacaatgtttaaaaaacccaattaacatttttacacaatttgggttctatttaaaaaaaaaaactggctctatctttaaatatggagcctaaccctgattcataaataccgtccctcttgaaaatggtcttcagttcaggcttctcatacctctgtgaacctagaattagaacaagtcatttcccttcccgtggccaacaagcatctagttgggaaccagtgatatcatcactgaacacactaaatacactgaggaaaattttgactgccatttaaccaaaaggctgcgtgatttcttcatttccctagttgaatggcaataaaacagctgccaataaaatctgcatggacacctacctttggttaatggtattgtaccacataagagagagcatcaccctcatcaaaacaaagtcaaatgagatcctctgctatacaaagagccctttaaaaagttataaatactaattatcaattacctttaaaatttctcagctgccagctctatcctatagggactttctgactgattaatcaggtcaaaagaatattgaccttttaactgtgctggagtcagcaaattcaacttgcatacacctttctatattaccaaacaatttcctcccgagggaaaagtgacacagtaacatttctgtgaggtgcaggcaaaaccaatgattcagtaatattaatattataacatcagacgaacagaattagttgattctgattctttggtggaatttccaggctgaagattcaaatctgaaggctcatcctgaggaaatataattttatcaggcgtataatcattcctcttcagatctggaagtttaagctttctacagcaagaattacagtgatgttttgctctgaagtttttaattgcatcttctcctagatttgctgggccaaaaaccatatcacaggatctcttttcttctgcttttatcacagatgggtcagtcaaattttcaccaacaccttgcaaatcaagtaccagtaactcccctcttgtatattcgtaagtccagtggctaaaggctagcatgatctcttccagagtattagttggaataatctcatctccattattattgttgtattttctaaattctccagtcatacattcttccacagcaaaccactgtcctgctgaatggcaatacagcaggaaaacttcaaggaaccttggagaatatggtatggatttgggtttcatttgattaaaggcaaacgtaagcttttgtgctgctctctgttgttgaatttctctcagacagagatgcagaactgtatcttctttgtaaatacttgaccatgtattaaccacctctggaagaaaagatttgataatataaagatgccctgatttgaggatatcatgttctgaccaggtacactgtactttgacagctcttcgtaaacctcctcccatctcctctttgcttaaaaactctattttggcacagaggcctagttgtgaccaagaagacatgctgttatttagtatgttgggtgaactctcttccaaacgatacactgtgacaggctcccctcttggaggcacaggtgtaaatggaatgctctgtgataacctcatcaagttatttctttccacagctgaataatagtaatttgtatccatagctggcttaaatggagaagtgagaccatttaatgttccttcttcagatggcatttctctgtttgatggtctatcttgtaaccaatccggtattaaagctgctttggaatctacttcatgagtgtcttcggtagatggccttctactgattttttctgcttgttttgaatgaacaggaatggaagttctgtgacagtcagtaaatccagcaagagaactcactcgtttcaaagtgttttcagaagtattgttattggatagtatttttatcttgtttgatgtttctttaaacctctgtaaatccatgctatctctgtgtcctacaaatgctccaaattctgtattatctccttctgtagctttagagcaaacagtttcttgatctttggttccagtttccaagtggcttttgcaacttggctgagatggtgtactaacaaaaaatttggttggtggggatgacagatgtggtatgctagtagatgaactgcctaatttttgatttttattaaatatttttaagagttctaccccatgtagtctctgtcgcagttctggaggggaaacagcacttgggaataaggcaccagaagaggaaccagcctctggaaaattaaattcttttctctggggtactgcaggtaagtcttgaccaaatatattacactggggatctttgtcatctttcattaaaatattacaatgaaaaggattattactttcaagatcaccttgaggaagagaggagctaagtgtatttacaacaccatgctttttccatacagaaggtcttacaggaccatcatcaataaggttttgagccaagtgtttggaaatgctcagttctcgtgtgatttcattatgaactttgctagcttccgacgctttctgggcagtgagtgtttttaatgtatctaccgtcagggctgaaagatcttgcaaatggccaatttgagaatctaatgattgtaatgatctttttatgtagttgacacgatctccaacttctttaatctgaatgcacatctgttccactctttcaaaagtgacacgaattctctcttcactcccagaatgaaatttgtcatctttttcattgaaatacatttcaacacactgctcttcaaaatcatgaagtttcttttgatcttcttctgttaagaaaagttttggtccatcggaagtcttatctttctttcttctcttacatatgcagcaaaacagagaaactatatggctaagaatgataagtggaggaggcagaactggtttctcatgataagccataataaaatgataacgctggtacttccatacaatattggaaattgccttcacttgtaaatacacattgttgaaaaatgcaataagaagattaaccataatgatatactgtacaaagaggtagactgcttgaagaaatggagtcaaccacgtcccaggaccacagatttgagggataacagaatcatttgcacacacatcaatttcgtatgcataaacttcaccaaaaatcatccagtatgggtgaaaaactatatctttagcaagagtccaagatggtgcttcatgaggataaagtattgcctttctgggaacaccaaaactaagtaatacaagagccataatcactacaatgtagaacatattggccaccatttttccaatcatcattacataaggtcctgcctgttgatttacagctagaaaatctagcaaacgcacataccaaaatattatgttaagacagtaaattaatcttccagccacaaaaacatgattatcatatgcatttgcaaagttccattttgctccaaatcttagtccaaatccaatgaagaaagaaattatggcaattgtatcactgatgttgaagtaatcactaaaccatactttaatcttctggtttactttcccagcttcagacataaagatctcacggactttctcaatggcataagtaaaaatataagcaataacaatccattcttgaactgaaggtaactgttccatttgtacaagaaccacaaatgtataaagcatcagaaatcctaaatatgccaacgtgttaaaccagaattttacaattggtgcatgataaaaggcataaaactttcgcgtaattggaagcttttttgatttcatttgtatctccatctcattctttccttcattactatccaaaatccgtacttctttaaacacttccatggggatctcttctgttatgttctgaaagttgttttcgctgtcatccattgtcatctgatgagcatcttgagattgtgggatatgggacatttcagccttagttttatactctaacagcaatatggcaggtggaactaaaatgcttagtatgaccttgtaccaggaatttttcctcatattcagccttcccatccacatatcagataacaacatttgtgtacaggtgtgagctacaaaaggtctaagtcttgaagaaactgctaacttaaggcaggttgaattactccagttcttcagttcataagtgagcaatttcatagccatggtttcatcttgtctgaaggactgttctaataattcaacggccaactgaccaaaatcattggaatactgttttagttcttctgaagtatcatctaccaggtcactctgctttgcttcatatgccattgaacgatagatcttacaggcaactaatgctttagccattgattcttcaccatgttgccataaaaaacgggccatgacctgcctcttcataaggcaagcccaaattaaaagttcattaagtggataaggaaagcgcttggtttctggatcatcaatgtctacaatttcatctttggttcttttcttctttccttcttccataactgtatcaatctttggtcggtagggctgtgctgtcttaatgaaatggttatgcctcattttttcctttttatctgccctattgccaaaagattcatgactctttcgcaactgaggagtgctgctggaggtatttcggccagacctccgattatttccaccaagactattatatattaatcgaaaacgtttcctagtataggtgcatctgtaggttcctcccatgagatattcaataacaagtcctatatcaatcagagtgatcttatatcctggaggaagatttccctgtttgacgtctcgaacaagatgaaacagcattggattagttggaccttgtttagtgttgtaaagttcttccagtctcggaatggtaaggaatttatgcatgcttactccattttcaataagaagttttacaaatgcaactctatccattacaagagcatcaagcatagcttgttccaaggatccaaccagccactgctgtccataaacaaatacatgatttttggcaatgtcaactctatcccatgccaatgtaaggataagctggtcaaatgcagatgcattagtaccttttagcagtgcagtaagtattgctacatctatatcttgatgttcatctgacccaatatggaaaacagtgataagctcctttcttttcatgcactccatcagtgtttgaaataaatgaagtgcttcattctggccaaagttaaatgtttttttgatagtggaaataatatcgggctctgctgcatcaggaagattccctccttcttctgtttgtttatgaatatacgctagcagatctgcagctctgcctgttccttcacacacaactactggaacaggggggctttcctgaaggtattcaagaactgtgaggataacatttggcccaccctcaaatataagtgccaccacagggacaccctggccaatcctagcatgaattctttgctgattaatagttttttcaagttctcttctcagtctgacttccgccccatactttccaacagtgccatcatccaccaatatgaaatgggaatgcagattattcaaaacattcaatttgctcagggggttcaataaggtttgataaggagcaaccacatctctcccaacaagatcatttctgttttcaatcactccccatggagctattccgatagtgcaaatctttcgagatgatctggaagcatgttctttgagggcatctccaacatgttttgccacacctgtgtttactcctccagttaaaatccaggctccagttgtaactgcagctttaataagaccttttccaagcaactgcttgattcgtgggtgaagctcaaatttctgcatgcccccatgtacagagataacaagtttgggtaactccatttgccattctttaagcagaagttgcagaatgacttcaggtttggtgtcatatgatagcctcacatacttagctctgtaggaatgagaacccccttgaaaatttatgactccataagcatccgttgggctctgttctgtatgcttttccacagaccattcttctattgcctgattaaaatggtcacccaatttcacatctgagtatttcatggcaagacttgcagtaaaacaagcatgttgcttgaccaagcgaccacaaaaacacctgacgagttgctgacaaatttgacatcctggaaggcatctgtgagggtccttggaacttggtataatatatacacattccctcttggtcaaagtgctttctatccaggatttctgggacattctcctcacggggcggactccggaagggcagcaactccacctcctcctcctccgcggcctgtagccatctatcgggaagcgtctccggaggcggcagcagaggccgccggacaaggaacgcccagggaaaccttctcagaactaactcagctccggcgctagcagcagaagccgagtctttcataattgtgcgaccaactcctccgggtgactggccacagggacgcgcccgcgcccgcctccgccggcgacggggctggggac

SEQ ID NO: 13740 - RNA, 8079 nt, Homo sapiens
  source 1..8079: mol_type = other RNA
gctgggattacaggcatgagccaccatgccccaccaagacaaacaaaacaaaacaaaacaaaacaaaacaaaacaaaaacagtatagatgaaaggcagccagcctgggttcaaatcctaccgttgctacttattattaaataaacgtaagaatcttatggacgttactttacctctctagcaccttgactttcaaatctgcaaaacaggataataacacctatttctttataacattgttataaggattaagtaggttaatatatgtgaaatacttagagtaatgtctggtacacagtaggcactaaataagtgttagcagccaggtgcggtggctcacaaggtcaggagtttgtgaccacactggccaacatagtgaaaccctgtctctactaaaaatataaaaattagctgggcatggtggcgtgtgcctgtagtcccagctactcgggaggctgaggcaggagaatcacttaaacccggaaggcggcggttgtggtgagctgagatcgcaccactgcactccagcccaagcaacagagcgagactccgtctcaaaaaaaaaaaaaaaaaaaaaagtatagctactattataatcctgtgaaaataatcaatataaaattaaaaatcaacagacagcccatattgcccttttttggcctaacaaaaaacagatttctaagaagacagtaagaaatcagtattaatttaaacattgtacaggacaggagatcaaaagcacaggtatacaaatggttcatttaaaaaaactgatactcaaattgacaccctgaaaatgtcagataatttttcagaatgattaaactcactaaacatctgtaaacaataaatttatttcatttcttttaaagatttaatgatatacaaaacgtatatagtatctttaagtaatacactttttctttctccccacccccaatcaatattaaacactatttaaacagcttatcatctcttgccttgtctgtatctatgagatacactactaaatacaaataagctttatactgctcccttccaaataaaaattaaaattagtaccaaggaaacaaaagaaaaagaaaaaaaaagaaaaaaaattaaagcataaaacttagatgaaaagcttttcttgttattgttgaatattcaacaatatctggggctgttaaattacattttattggcataaggttgcactgcaatctgccagtatcacataatgataatccaactgaattaatttcttaagtaccacaaacagcattcatgttcaaatgttccaacacaattttaaatatatgcaagagttcatgtttacattctgatttgatataacaatcaataaaatctttggagaagtttgtaagttctgggttgttgctatagatacagatagggaaaaaagtactttaactttcctcaaaaggtaacttcccttgacgagtgagttaggtttctgcttttataatttaggttatgtatcagtttaccatggctttcttctacttaacagtgacttgataaaacaatgtttaaaaaacccaattaacatttttacacaatttgggttctatttaaaaaaaaaaactggctctatctttaaatatggagcctaaccctgattcataaataccgtccctcttgaaaatggtcttcagttcaggcttctcatacctctgtgaacctagaattagaacaagtcatttcccttcccgtggccaacaagcatctagttgggaaccagtgatatcatcactgaacacactaaatacactgaggaaaattttgactgccatttaaccaaaaggctgcgtgatttcttcatttccctagttgaatggcaataaaacagctgccaataaaatctgcatggacacctacctttggttaatggtattgtaccacataagagagagcatcaccctcatcaaaacaaagtcaaatgagatcctctgctatacaaagagccctttaaaaagttataaatactaattatcaattacctttaaaatttctcagctgccagctctatcctatagggactttctgactgattaatcaggtcaaaagaatattgaccttttaactgtgctggagtcagcaaattcaacttgcatacacctttctatattaccaaacaatttcctcccgagggaaaagtgacacagtaacatttctgtgaggtgcaggcaaaaccaatgattcagtaatattaatattataacatcagacgaacagaattagttgattctgattctttggtggaatttccaggctgaagattcaaatctgaaggctcatcctgaggaaatataattttatcaggcgtataatcattcctcttcagatctggaagtttaagctttctacagcaagaattacagtgatgttttgctctgaagtttttaattgcatcttctcctagatttgctgggccaaaaaccatatcacaggatctcttttcttctgcttttatcacagatgggtcagtcaaattttcaccaacaccttgcaaatcaagtaccagtaactcccctcttgtatattcgtaagtccagtggctaaaggctagcatgatctcttccagagtattagttggaataatctcatctccattattattgttgtattttctaaattctccagtcatacattcttccacagcaaaccactgtcctgctgaatggcaatacagcaggaaaacttcaaggaaccttggagaatatggtatggatttgggtttcatttgattaaaggcaaacgtaagcttttgtgctgctctctgttgttgaatttctctcagacagagatgcagaactgtatcttctttgtaaatacttgaccatgtattaaccacctctggaagaaaagatttgataatataaagatgccctgatttgaggatatcatgttctgaccaggtacactgtactttgacagctcttcgtaaacctcctcccatctcctctttgcttaaaaactctattttggcacagaggcctagttgtgaccaagaagacatgctgttatttagtatgttgggtgaactctcttccaaacgatacactgtgacaggctcccctcttggaggcacaggtgtaaatggaatgctctgtgataacctcatcaagttatttctttccacagctgaataatagtaatttgtatccatagctggcttaaatggagaagtgagaccatttaatgttccttcttcagatggcatttctctgtttgatggtctatcttgtaaccaatccggtattaaagctgctttggaatctacttcatgagtgtcttcggtagatggccttctactgattttttcttgttttgaatgaacaggaatggaagttctgtgacagtcagtaaatccagcaagagaactcactcgtttcaaagtgttttcagaagtattgttattggatagtatttttatcttgtttgatgtttctttaaacctctgtaaatccatgctatctctgtgtcctacaaatgctccaaattctgtattatctccttctgtagctttagagcaaacagtttcttgatctttggttccagtttccaagtggcttttgcaacttggctgagatggtgtactaacaaaaaatttggttggtggggatgacagatgtggtatgctagtagatgaactgcctaatttttgatttttattaaatatttttaagagttctaccccatgtagtctctgtcgcagttctggaggggaaacagcacttgggaataaggcaccagaagaggaaccagcctctggaaaattaaattcttttctctggggtactgcaggtaagtcttgaccaaatatattacactggggatctttgtcatctttcattaaaatattacaatgaaaaggattattactttcaagatcaccttgaggaagagaggagctaagtgtatttacaacaccatgctttttccatacagaaggtcttacaggaccatcatcaataaggttttgagccaagtgtttggaaatgctcagttctcgtgtgatttcattatgaactttgctagcttccgacgctttctgggcagtgagtgtttttaatgtatctaccgtcagggctgaaagatcttgcaaatggccaatttgagaatctaatgattgtaatgatctttttatgtagttgacacgatctccaacttctttaatctgaatgcacatctgttccactctttcaaaagtgacacgaattctctcttcactcccagaatgaaatttgtcatctttttcattgaaatacatttcaacacactgctcttcaaaatcatgaagtttcttttgatcttcttctgttaagaaaagttttggtccatcggaagtcttatctttctttcttctcttacatatgcagcaaaacagagaaactatatggctaagaatgataagtggaggaggcagaactggtttctcatgataagccataataaaatgataacgctggtacttccatacaatattggaaattgccttcacttgtaaatacacattgttgaaaaatgcaataagaagattaaccataatgatatactgtacaaagaggtagactgcttgaagaaatggagtcaaccacgtcccaggaccacagatttgagggataacagaatcatttgcacacacatcaatttcgtatgcataaacttcaccaaaaatcatccagtatgggtgaaaaactatatctttagcaagagtccaagatggtgcttcatgaggataaagtattgcctttctgggaacaccaaaactaagtaatacaagagccataatcactacaatgtagaacatattggccaccatttttccaatcatcattacataaggtcctgcctgttgatttacagctagaaaatctagcaaacgcacataccaaaatattatgttaagacagtaaattaatcttccagccacaaaaacatgattatcatatgcatttgcaaagttccattttgctccaaatcttagtccaaatccaatgaagaaagaaattatggcaattgtatcactgatgttgaagtaatcactaaaccatactttaatcttctggtttactttcccagcttcagacataaagatctcacggactttctcaatggcataagtaaaaatataagcaataacaatccattcttgaactgaaggtaactgttccatttgtacaagaaccacaaatgtataaagcatcagaaatcctaaatatgccaacgtgttaaaccagaattttacaattggtgcatgataaaaggcataaaactttcgcgtaattggaagcttttttgatttcatttgtatctccatctcattctttccttcattactatccaaaatccgtacttctttaaacacttccatggggatctcttctgttatgttctgaaagttgttttcgctgtcatccattgtcatctgatgagcatcttgagattgtgggatatgggacatttcagccttagttttatactctaacagcaatatggcaggtggaactaaaatgcttagtatgaccttgtaccaggaatttttcctcatattcagccttcccatccacatatcagataacaacatttgtgtacaggtgtgagctacaaaaggtctaagtcttgaagaaactgctaacttaaggcaggttgaattactccagttcttcagttcataagtgagcaatttcatagccatggtttcatcttgtctgaaggactgttctaataattcaacggccaactgaccaaaatcattggaatactgttttagttcttctgaagtatcatctaccaggtcactctgctttgcttcatatgccattgaacgatagatcttacaggcaactaatgctttagccattgattcttcaccatgttgccataaaaaacgggccatgacctgcctcttcataaggcaagcccaaattaaaagttcattaagtggataaggaaagcgcttggtttctggatcatcaatgtctacaatttcatctttggttcttttcttctttccttcttccataactgtatcaatctttggtcggtagggctgtgctgtcttaatgaaatggttatgcctcattttttcctttttatctgccctattgccaaaagattcatgactctttcgcaactgaggagtgctgctggaggtatttcggccagacctccgattatttccaccaagactattatatattaatcgaaaacgtttcctagtataggtgcatctgtaggttcctcccatgagatattcaataacaagtcctatatcaatcagagtgatcttatatcctggaggaagatttccctgtttgacgtctcgaacaagatgaaacagcattggattagttggaccttgtttagtgttgtaaagttcttccagtctcggaatggtaaggaatttatgcatgcttactccattttcaataagaagttttacaaatgcaactctatccattacaagagcatcaagcatagcttgttccaaggatccaaccagccactgctgtccataaacaaatacatgatttttggcaatgtcaactctatcccatgccaatgtaaggataagctggtcaaatgcagatgcattagtaccttttagcagtgcagtaagtattgctacatctatatcttgatgttcatctgacccaatatggaaaacagtgataagctcctttcttttcatgcactccatcagtgtttgaaataaatgaagtgcttcattctggccaaagttaaatgtttttttgatagtggaaataatatcgggctctgctgcatcaggaagattccctccttcttctgtttgtttatgaatatacgctagcagatctgcagctctgcctgttccttcacacacaactactggaacaggggggctttcctgaaggtattcaagaactgtgaggataacatttggcccaccctcaaatataagtgccaccacagggacaccctggccaatcctagcatgaattctttgctgattaatagttttttcaagttctcttctcagtctgacttccgccccatactttccaacagtgccatcatccaccaatatgaaatgggaatgcagattattcaaaacattcaatttgctcagggggttcaataaggtttgataaggagcaaccacatctctcccaacaagatcatttctgttttcaatcactccccatggagctattccgatagtgcaaatctttcgagatgatctggaagcatgttctttgagggcatctccaacatgttttgccacacctgtgtttactcctccagttaaaatccaggctccagttgtaactgcagctttaataagaccttttccaagcaactgcttgattcgtgggtgaagctcaaatttctgcatgcccccatgtacagagataacaagtttgggtaactccatttgccattctttaagcagaagttgcagaatgacttcaggtttggtgtcatatgatagcctcacatacttagctctgtaggaatgagaacccccttgaaaatttatgactccataagcatccgttgggctctgttctgtatgcttttccacagaccattcttctattgcctgattaaaatggtcacccaatttcacatctgagtatttcatggcaagacttgcagtaaaacaagcatgttgcttgaccaagcgaccacaaaaacacctgacgagttgctgacaaatttgacatcctggaaggcatctgtgagggtccttggaacttggtataatatatacacattccctcttggtcaaagtgctttctatccaggatttctgggacattctcctcacggggcggactccggaagggcagcaactccacctcctcctcctccgcggcctgtagccatctatcgggaagcgtctccggaggcggcagcagaggccgccggacaaggaacgcccagggaaaccttctcagaactaactcagctccggcgctagcagcagaagccgagtctttcataattgtgcgaccaactcctccgggtgactggccacagggacgcgcccgcgcccgcctccgccggcgacggggctggggac

SEQ ID NO: 13741 - RNA, 1855 nt, Homo sapiens
  source 1..1855: mol_type = other RNA
gctgggattacaggcatgagccaccatgcccgaccataatttcctctcttttaaaccttagatttgaatgatttttgctggattcttcaaacatgaagtattttttaaattgaaaactaattgaatgactttaactggtaagtagaagtcttagaccgttgactaaaagctaaggctaacgttgaccctgcaaaagggggccactgaaggcccagttgattattcctgggtgtctgccctgcagacatcaaagtctgctcacaccaaccatagaaggagcctttgtcactgtcagaagatacagagctttggtaagctggaagttgacaggcagatgcagttggggttgagattgaagaaaagttgggatattctttctagaatggagttgttattgtcctgagactgtttatagactttgtctaagaagttacttaagaagtgttgtaacaaggaaaaagtacaaatgattagatctttgaggatctcaaaggttaggtggaaaagggttttatttcatagggaggagaaaataagtttacaaagaaggttggaaaggaagcacaggatggagggtagcaaaatcagatcccagataagataatgtttcatcttgaagtcagcctgttcttaggagggatatgtataaatatgggttgtaggttctctgaggctgtgggtgagtcaaagttcaggggctctagccaagtgcctgggatggatcctttctgcgtctcaccaaggctcaccacttagccatagcctcaaacccgtggggaaggaaggtctccccgccctgagacttagatgacaggcctgcagaacttggttctctctatagtccctgaatcaggcaaaacacaccttctttccttctccagccatggtctggaagaaatcttcacattgatatgatgaaatgctaactaacaatatgaaaaatactaaagtataaatgtcactaaaatggtaaatacatactgaatttcagaatactataaattgttatcatcttaaactagactattaaaatacaagatgttttacataagtctcatgataaccagtaggaaaaaaaaatagtaaagaaaaagagaaagtaattaaagcatacacaaacaacaaaaattacacattggatatggtgtctcctgcttataattccaacactttgggaggccaaggtggaagaatcaaatctccttgggtgttgtggtacatgtctgcagtccaagctacttgggtggctaaggtgggacgattatttgagcccaggaggttaaggctacagtgagctgtgatatgccactgcacttcagtctgagcaagaaagcataactttgtctcaacaaaaatgaacaataccacaggaaagacagaaccagaaaaaaaagaagcaaacttaaaatggacagaaaactacaaatgtacaatagtaactgcttacctatcactaccttacaaataaaaagattaaagtatctactaaacagatactgctgtacactgaatgtcatctccaaaatttaggataaaatttaatagccaacatgttagaattaacaggtggaacctttaaaaattaattaagctataagcactctgccctcatgaatggattaacgttcttattatgggaatgggctaattataacaagaatggatctgttatatattaaaaaaaaaaagctctctctccctcacatctttgtgtatgttattatccagcaactagaccttcaacatataccagtataatgttgttttggcttcccagcctccagaatcatgagtcaaataaaattctattctttattaattaccagtgtgtgatattctgttatagcagccaaaa

SEQ ID NO: 13742 - RNA, 3160 nt, Homo sapiens
  source 1..3160: mol_type = other RNA
gctgggattacaggcatgagccaccatgcccgaccataatttcctctcttttaaaccttagatttgaatgatttttgctggattcttcaaacatgaagtattttttaaattgaaaactaattgaatgactttaactggtaagtagaagtcttagaccgttgactaaaagctaaggctaacgttgaccctgcaaaagggggccactgaaggcccagttgattattcctgggtgtctgccctgcagacatcaaagtctgctcacaccaaccatagaaggagcctttgtcactgtcagaagatacagagctttggtaagctggaagttgacaggcagatgcagttggggttgagattgaagaaaagttgggatattctttctagaatggagttgttattgtcctgagactgtttatagactttgtctaagaagttacttaagaagtgttgtaacaaggaaaaagtacaaatgattagatctttgaggatctcaaaggttaggtggaaaagggttttatttcatagggaggagaaaataagtttacaaagaaggttggaaaggaagcacaggatggagggtagcaaaatcagatcccagataagataatgtttcatcttgaagtcagcctgttcttaggagggatatgtataaatatgggttgtaggttctctgaggctgtgggtgagtcaaagttcaggggctctagccaagtgcctgggatggatcctttctgcgtctcaccaaggctcaccacttagccatagcctcaaacccgtggggaaggaaggtctccccgccctgagacttagatgacaggcctgcagaacttggttctctctatagtccctgaatcaggcaaaacacaccttctttccttctccagccatggtctggaagaaatcttcacattgatatgatgaaatgctaactaacaatatgaaaaatactaaagtataaatgtcactaaaatggtaaatacatactgaatttcagaatactataaattgttatcatcttaaactagactattaaaatacaagatgttttacataagtctcatgataaccagtaggaaaaaaaaatagtaaagaaaaagagaaagtaattaaagcatacacaaacaacaaaaattacacattggatatggtgtctcctgcttataattccaacactttgggaggccaaggtggaagaatcaaatctccttgggtgttgtggtacatgtctgcagtccaagctacttgggtggctaaggtgggacgattatttgagcccaggaggttaaggctacagtgagctgtgatatgccactgcacttcagtctgagcaagaaagcataactttgtctcaacaaaaatgaacaataccacaggaaagacagaaccagaaaaaaaagaagcaaacttaaaatggacagaaaactacaaatgtacaatagtaactgcttacctatcactaccttacaaataaaaagattaaagtatctactaaacagatactgctgtacactgaatgtcatctccaaaatttaggataaaatttaatagccaacatgttagaattaacaggtggaacctttaaaaattaattaagctataagcactctgccctcatgaatggattaacgttcttattatgggaatgggctaattataacaagaatggatctgttatatatttaaaaaaaaaagctctctctccctcacatctttgtgtatgttattatccagcaactagaccttcaacatataccagtataatgttgttttggcttcccagcctccagaatcatgagtcaaataaaattctattctttattaattaccagtgtgtgatattctgttatagcagccaaaagagactaaagcagacagagtggataaattaatcttttaaacctcataatatgctgcttacaagagactcaattatgaattaagagcataggctaaaagtgaaaggatagaaaatgatattccatgcaaataataaccaaaggagtgaaatggtaatgcttaaattagacaaaatagactttctagcaatgtctctcacaagaatgaaatgagtttaccatacaataatagaggttaatttctcaagagaatatagctttatatatttatgcacccaaaagggaggcttctaaatataaaaagcaaatattgccagaactgtagggagaagtagaaagaaacccaataatagaaaactttaacgaaatgtataataaaggacatatagttaacagcattgtaaattggcaagggaaagctggtctcatgtgttgcgtttgagaatgcagcaaagaaagtgggaactgataattttactgcaagcctgagttaggatgaaaaacagggtggtcgattagaggttccacttgccatacattaaaaaaacacaggagaaaaccagtcctcctctggagtgttaaaataattaaagatcagaaaattagtctaaagtggctctagtgccctgtgttcataggtaaaaaacaaaaaacaaacaaaaaaaaatctaaaacctaactcaaatatatttcctataaaacactatcttagcctgaagcaaaatgcaggtttaacccatgacaaacatgcaattaacctctgaatatgtaaccaggacatttccatctggatagttcaaataaggctaccatataactggaaccaattcttgaatttgggttgctttctcatgcatcttatgaaagcctttcctttatgcccctctggtggaccagaaatcatggctgggtgctttccatttcaccaatcactctttgttcagataaactgatgaaccttttaacatagactcccgttaatttttaacacgagagactgtggaccccacgggccgcagctcctcccacgcaaacacccactcgcggtttttccctgatgacccatctggcctccctgaacaatttgggaaatactcatggctgtgggcgcagagcagggcgctgcccagggacaggaccggatgggccggacgggacgtgggggtcctcgctgctggcccagcggccatcttgcagccacaggggactgagggccaagctgcgggagactcggagctaaccgtggggaggccggtcctgccggtttcacagtctgttctcccctctcgggatggcgaaccccgtat

SEQ ID NO: 13743 - RNA, 4831 nt, Homo sapiens
  source 1..4831: mol_type = other RNA
gctgggattacaggcatgagccaccatgcccgacttccctttgtgtaaaatgagataatatgtatgtcacagaattgttttaaggatgataaaggactaagtgagataatgtaggtgaagtttagtatgatgcctggctcatagttaagtgctgaattatgatagtaatcaatatctactcctaacctctttcttcacagattttaagcttctgtctttctagggggttaagagtcataaaccaaaattacactttcctctgctaggtttcctccctttcctcttcttgacagtctgatgggaaacaaaggcacacataagagcctagttccaagtagtcaagagcctgagaggaagggatatggagagtaatccttcatatctccaggagtgcctgtgaagaagctgaggaatgggactgggaaagcacacaaaataaggaaaacctttcctggggttgggaaagagaagaaagtgcacagctggctacataccataagaattttgtgtcaaaatgtttaaaagcctccaaagattgaatggaattgtctgggactggggaaaaggggctgggacctgggagagagagggaatagggagaagacggtaccctctaaaggcactagctgccattaaatgctccctgagtgccacagggagcaggagttacgttctctgggcattagccttggggaaaagcctgctatgccagtaatcagggttatcaaaggcagagtctgtagcctctaagctacgtagagtttttaggcgggcataatggacatggggggcctgatgtccaggcccctgaaaagctctcatctcttcatacccttgctcagatgctgggcaggcccccatggctgcataatcacccccaggaccacctccatctcgttgccgattcatatattcatagtcttcatctggagttgtgcctgcagtgggcatgatgggtacagggtggagtgggcaactctgtgtgctgcccagagaggcactgaggtctgaccccacatccatgtactcataacccagctcctcaagggaacttggcctagggggatgaggtggactgtgccttctcctccggttcatgtattcatactcctcatcttcatcttcttcttcagtacccaggacagaactgagacccactgaagaaagggtgccttcccgggaggagggagtacctttgaggtgtgtatctggcatgacataaccgttgacatcctcttcctctaacccgggtggggagagtggggtaacaggagtcagcagactgtggcgctgggaatggtaggcgctatctccgcgtggccgtgggctccggctcctgctccggctcctacacattgacactttctcctggagctcagcctcagagcctgttacatgcccctctgatgactctgatgccaggcatccccgtggcattgggtgtagagagactggacgggggcaccgttcactgctcccagaaactgcagactcctggcaagactccccaagattaccctggttcatgggcatgtatccagatgatggacttaaaaggctctggctcccacgtggccgattaagtgttccaactggtaggctgagggcggagcccagtgtggtggttgccaggttgtcctcctctgcttccaagtctaggtctaggtctagttctggctccagctctacttcctctagcttcttgtttgtcagaccatggggctctggcccaggggctattccaggcccactctctctctttatgaccagataccgtggtgggtctcgggccatcctggtgaactcattggctagttctttaaaggttgggcgaatgttctcatcaatcatccaacacttgaccatcaccatgtagacatcaattgtgcagatctggggctgtgccaaccgctcccccttctctagcaggtctggtacttcagccaatcgtagccctgcatagggctctgccccgaaggtcatcaactcccaaactgtcacaccatagctccagacatcactctggtgtgtgtatttcccaaagtggatactctcaagggccatccacttaattggagtcttggcctcactgtatagcagctgcttatcatcaggaggcagcaggtcagccacaccaaaatctgccacctgaacctgactgggtgacttgagtagcacgtttcgggcagccaggtttctatgcaccataccatgttcctcaaggtagtacattcccttggcaatttgtactccccagttgagcagcagctgtggccccagtgccccccggtgttgtctcacatgatccagcagagaacccagaggcaaatattgagtgacaagctgcagagatgaccctgggcatagtcccagcagccttacaatgtgggcatggtccaggctgccaatggccagcatatgatctgtcacagcttgaaaactctgccgtccactcttgtcctcaatgactttaatgcagactggaatcttgattgattcaccctcagggatccacactcctttgtgcacagttccaaagacacccgagccaagcactttaagcttccttagctctgtctctttgaagattctggccaagactttgttagccttctcactggggtccagaggctctatgctctcaccccgttccaagtatcgcctcatagcccttttattctgaatccggcgcccacgccagtagagaaaagtgccgcccagcatcatgaaaatcactaccaatcctgctatcactgtcaaagccattgtcagatgggttttgccgatcagcaccagtgtttgtcctaaacagtcttgaagctctggtcctttacacccctgggtgcagttctcatggcagggccgacattcattctgaacatctgggtacttgtagattgggcccttggcacctaggactccatgggggcagctgctcacacagtggggcccatctcgaaaatgggcacattgagcacaagtatcagagcccgagccattgcatgtggcagtgccctccatgggttggcattccgggtggcaggagaagcattcggcctcatgggcaaattctcgaggctccccattcagaaagttgcagtgggtcacacagacacctcctcggctataatttcgacaggacaagcactgaccagggcctgggccccagcatcccccagaggagcacagtgggtcacacactttgccctctgccacgcagtctctgcgcggccgattatgcttgatgtctagtcgctcttccgtaggcccccgaagcaccttggtccagttcaaagagtggtggtagcagagctgcctattggcacttatatagatacgcccagcactaatttccttcagggatcggaagcccagagatgtgacattcaagttcttcatgatcaacaatgagaagccccggttgtagaggcttctgcctccaatggttgtcaaattggaaaaaacactgaagttgtgcatgtggggcggccaggactggatgttcaggtaacctgtgatctcccgtactgtccggaagacattgagcttctctgggtccagggcagggatcttgtgccaggggtctccattgaggccggtgatcagaaagtccaggttgcccaggatcttggtgcagttcacaaatccatcaatgttgctcgagtccacagtctggaagcggctcccagagcctgttccctcacaggctttgggacatagtcccccacaaggctcacacatcttgagcccatttttatctacttccatcttgtcaggaggacaggccctgacacaggatgtttgatccaccacaaagttatggggacagctggctacacaaactcctccatactgatacttggtgtggggattgggttccagctggaaagttagcttgttgtagacaagaggctgtggacagcgaggtacacaggctccactgtcattgaagtgccggcaggcaaagcagtctgtgtcctgagggcctgagcagcccccggcacactcatcatggcagcactggttggggttgggcccaaagcagtgaccattacactgaggagcacagatggtcttggtcaatgtctggcagtcttctgatccaggaccccagcatcgccccttgcaaacctcatgacaggggggacagcttctgccattgtccttcaccactatctcagcatctcggtccctcacgatgtccctccagtcaattgtgtccatgtgacaaagcttatcgttcttctcaatataaacaccccctgacagaatctcggtgagctgagtcaagcggagctggcgcagagcgtggctggagttggtgttatagttcaacatgacgaagatggcaaacttcccatcgtagacctgggtccctcgcaccacgcggaggttgggcaatggtagagtagagaattcattcatggccacgaggacatagcctgtcacttctcgaatccactgcaggaaggagaggtcggcattgtgtcccgtgagcacaatctcaaggttccccatcaccacctcacacctctcgtagagcttgtacagtgtctggtattggttctcagcatcgccggtcacactcaggccattcagagtcccaggacacactgcctgagagttgcccacctcggagccccgggccaggctgaaaagcaagcccagcacctgcagagcgtcgttcgccctcatgactccgcagagggtgaagggagcccagccaagtccggcccgggggcccctaggctaggacatcgaggcaagagccacctgaaccgctggcgaattggtggctgctgcggcgacggcagcggaggttgcaaattgc

SEQ ID NO: 13744 - RNA, 1411 nt, Homo sapiens
  source 1..1411: mol_type = other RNA
gctgggattacaggcatgagccaccatgcccggccaaaaaacttgactattcttgatgccaagacaagagaaacttaattatgacgttagaagtttcaaaaatacagtgacttctgggacacttctagtagccaaaaatccacagatgcccagaccccctccttctgcattccagaatcagatgtttacattccaagacagaaagaatctgaaacaacggcctacaagaaatttgggaaatgacatttgatctcattttcctctcaattggaagtcatgatatcaatgaatatcaaatggaaaaataagctcagaagtaggtgagaattatgatctctaaaacgcaggtgctgatttctaatccttctcataaaattccggatcacaaattgagggctgatgagaagatcttacaccgaaggcactaactggcactaatgtgagccagcaacatgtgaaaggctaatccaggagatgcagaaatgcacatgggttccaggtgtcttttctaagtgacaatgggcctccttactggacagtagtcaggagacaattcaaatgtacttaataaaattgtcaggtgggcaaccaaagggaagagacttaaaagacctcccagaactgggatggaaaataagccaaacactactagcagcaggaccagctggaggacttggtttgtagattgatgtagtccccttgggtggacaaagacatgatatcttctgtggaatttctcatcatcttttcaatgaggactctcatagcctcattaatatttttgttctccttgactgatgtttctgtccaacctgtgaaaccgttctctttactgaaccggtcaatctggtcccggctcactgcccaaggggacagatcacacttgttggccaagagcaggcagggcaccggctctccattgggtagtgtgagcttgctgtctaggtcctgtttccacctctggctgttgctgaaggtagtggcattggtaacgtcaaacataataacacaggcagaggcatcccgataatacaatcgtgtcatagaggtgaagcgctcctgccctcccaccgtggacttgtagtgtttgctgaagctgtcctgggaatatcgctgcaccagcgacgtcttgcccactgcggcgtcccccaccaccagcactttgaacaggtggtcgcggctgcccatggctagcggggtgtgcgttttagggaggcgggaagtgtggtcggggatcgggggtcgctcgttttaacccctttggatccggaccctcttcaaactgaagtgaggcattcccacccaccgcctgtctgggcaaattgtgaggaaggagcagccggcacctcgattccctagacgccctcccgcgcgcctctctctccccttcctccgcaagcgtcacgtgcag

SEQ ID NO: 13745 - RNA, 1501 nt, Homo sapiens
  source 1..1501: mol_type = other RNA
gctgggattacaggcatgagccaccatgcccggccaaaaaacttgactattcttgatgccaagacaagagaaacttaattatgacgttagaagtttcaaaaatacagtgacttctgggacacttctagtagccaaaaatccacagatgcccagaccccctccttctgcattccagaatcagatgtttacattccaagacagaaagaatctgaaacaacggcctacaagaaatttgggaaatgacatttgatctcattttcctctcaattggaagtcatgatatcaatgaatatcaaatggaaaaataagctcagaagtaggtgagaattatgatctctaaaacgcaggtgctgatttctaatccttctcataaaattccggatcacaaattgagggctgatgagaagatcttacaccgaaggcactaactggcactaatgtgagccagcaacatgtgaaaggctaatccaggagatgcagaaatgcacatgggttccaggtgtcttttctaagtgacaatgggcctccttactggacagtagtcaggagacaattcaaatgtacttaataaaattgtcaggtgggcaaccaaagggaagagacttaaaagacctcccagaactgggatggaaaataagccaaacactactagcagcaggaccagctggaggacttggtttgtagattgatgtagtccccttgggtggacaaagacatgatatcttctgtggaatttctcatcatcttttcaatgaggactctcatagcctcattaatatttttgttctccttgactgatgtttctgtccaacctgtgaaaccgttctctttactgaaccggtcaatctggtcccggctcactgcccaaggggacagatcacacttgttggccaagagcaggcagggcaccggctctccattgggtagtgtgagcttgctgtctaggtcctgtttccacctctggctgttgctgaaggtagtggcattggtaacgtcaaacataataacacaggcagaggcatcccgataatacaatcgtgtcatagaggtgaagcgctcctgccctcccaccgtggacttgtagtgtttgctgaagctgtcctgggaatatcgctgcaccagcgacgtcttgcccactgcggcgtcccccaccaccagcactttgaacaggtggtcgcggctgcccatggctagcggggtgtgcgttttagggaggcgggaagtgtggtcggggatcgggggtcgctcgttttaacccctttggatccggaccctcttcaaactgaagtgaggcattcccacccaccgcctgtctgggcgggacttcccccgagcggctccaagtcagtgactgaatcccagtcagctccttacaccactggggccagatgatggggaccctccccttgcagcacaaaccaaattgtgaggaaggagcagccggcacctcgattccctagacgccctcccgcgcgcctctctctccccttcctccgcaagc

SEQ ID NO: 13746 - RNA, 1479 nt, Homo sapiens
  source 1..1479: mol_type = other RNA
gctgggattacaggcatgagccaccatgcccggccaaaaaacttgactattcttgatgccaagacaagagaaacttaattatgacgttagaagtttcaaaaatacagtgacttctgggacacttctagtagccaaaaatccacagatgcccagaccccctccttctgcattccagaatcagatgtttacattccaagacagaaagaatctgaaacaacggcctacaagaaatttgggaaatgacatttgatctcattttcctctcaattggaagtcatgatatcaatgaatatcaaatggaaaaataagctcagaagtaggtgagaattatgatctctaaaacgcaggtgctgatttctaatccttctcataaaattccggatcacaaattgagggctgatgagaagatcttacaccgaaggcactaactggcactaatgtgagccagcaacatgtgaaaggctaatccaggagatgcagaaatgcacatgggttccaggtgtcttttctaagtgacaatgggcctccttactggacagtagtcaggagacaattcaaatgtacttaataaaattgtcaggtgggcaaccaaagggaagagacttaaaagacctcccagaactgggatggaaaataagccaaacactactagcagcaggaccagctggaggacttggtttgtagattgatgtagtccccttgggtggacaaagacatgatatcttctgtggaatttctcatcatcttttcaatgaggactctcatagcctcattaatatttttgttctccttgactgatgtttctgtccaacctgtgaaaccgttctctttactgaaccggtcaatctggtcccggctcactgcccaaggggacagatcacacttgttggccaagagcaggcagggcaccggctctccattgggtagtgtgagcttgctgtctaggtcctgtttccacctctggctgttgctgaaggtagtggcattggtaacgtcaaacataataacacaggcagaggcatcccgataatacaatcgtgtcatagaggtgaagcgctcctgccctcccaccgtggacttgtagtgtttgctgaagctgtcctgggaatatcgctgcaccagcgacgtcttgcccactgcggcgtcccccaccaccagcactttgaacaggtggtcgcggctgcccatggctagcggggtgtgcgttttagggaggcgggaagtgtggtcggggatcgggggtcgctcgttttaacccctttggatccggaccctcttcaaactgaagtgaggcattcccacccaccgcctgtctgggctgctcgggacttcccccgagcggctccaagtcagtgactgaatcccagtcagctccttacaccactggggccagatgatggggaccctccccttgcagcacaaaccaaattgtgaggaaggagcagccggcacctcgattccctagacgccctcccgcgc

SEQ ID NO: 13747 - RNA, 1714 nt, Homo sapiens
  source 1..1714: mol_type = other RNA
gctgggattacaggcatgagccaccatgcccggccaaaaaacttgactattcttgatgccaagacaagagaaacttaattatgacgttagaagtttcaaaaatacagtgacttctgggacacttctagtagccaaaaatccacagatgcccagaccccctccttctgcattccagaatcagatgtttacattccaagacagaaagaatctgaaacaacggcctacaagaaatttgggaaatgacatttgatctcattttcctctcaattggaagtcatgatatcaatgaatatcaaatggaaaaataagctcagaagtaggtgagaattatgatctctaaaacgcaggtgctgatttctaatccttctcataaaattccggatcacaaattgagggctgatgagaagatcttacaccgaaggcactaactggcactaatgtgagccagcaacatgtgaaaggctaatccaggagatgcagaaatgcacatgggttccaggtgtcttttctaagtgacaatgggcctccttactggacagtagtcaggagacaattcaaatgtacttaataaaattgtcaggtgggcaaccaaagggaagagacttaaaagacctcccagaactgggatggaaaataagccaaacactactagcagcaggaccagctggaggacttggtttgtagattgatgtagtccccttgggtggacaaagacatgatatcttctgtggaatttctcatcatcttttcaatgaggactctcatagcctcattaatatttttgttctccttgactgatgtttctgtccaacctgtgaaaccgttctctttactgaaccggtcaatctggtcccggctcactgcccaaggggacagatcacacttgttggccaagagcaggcagggcaccggctctccattgggtagtgtgagcttgctgtctaggtcctgtttccacctctggctgttgctgaaggtagtggcattggtaacgtcaaacataataacacaggcagaggcatcccgataatacaatcgtgtcatagaggtgaagcgctcctgccctcccaccgtggacttgtagtgtttgctgaagctgtcctgggaatatcgctgcaccagcgacgtcttgcccactgcggcgtcccccaccaccagcactttgaacaggtggtcgcggctgcccatggctagcggggtgtgcgttttagggaggcgggaagtgtggtcggggatcgggggtcgctcgttttaacccctttggatccggaccctcttcaaactgaagtgaggcattcccacccaccgcctgtctgggctgctctgacgagaaagcaaaaaaggaaactttgcactcaacctatacgcgcttcctccccgggcggccgcaacctgggtggggcgcagggcgcgagctccgagcccccggctgttcgcaccttccccaccccctcctggcctgactgccgagaaactggaccaggcgccgcggaacctcacccaccgggacttcccccgagcggctccaagtcagtgactgaatcccagtcagctccttacaccactggggccagatgatggggaccctccccttgcagcacaaaccaaattgtgaggaaggagcagccggcacctcgattccctagacgccctcccgcgcgcctctctctccccttcctccgcaagcgtcacgtgcagggttgcctgtggcact

SEQ ID NO: 13748 - RNA, 1242 nt, Homo sapiens
  source 1..1242: mol_type = other RNA
gctgggattacaggcatgagccaccatgcccggccaaaaaacttgactattcttgatgccaagacaagagaaacttaattatgacgttagaagtttcaaaaatacagtgacttctgggacacttctagtagccaaaaatccacagatgcccagaccccctccttctgcattccagaatcagatgtttacattccaagacagaaagaatctgaaacaacggcctacaagaaatttgggaaatgacatttgatctcattttcctctcaattggaagtcatgatatcaatgaatatcaaatggaaaaataagctcagaagtaggtgagaattatgatctctaaaacgcaggtgctgatttctaatccttctcataaaattccggatcacaaattgagggctgatgagaagatcttacaccgaaggcactaactggcactaatgtgagccagcaacatgtgaaaggctaatccaggagatgcagaaatgcacatgggttccaggtgtcttttctaagtgacaatgggcctccttactggacagtagtcaggagacaattcaaatgtacttaataaaattgtcaggtgggcaaccaaagggaagagacttaaaagacctcccagaactgggatggaaaataagccaaacactactagcagcaggaccagctggaggacttggtttgtagattgatgtagtccccttgggtggacaaagacatgatatcttctgtggaatttctcatcatcttttcaatgaggactctcatagcctcattaatatttttgttctccttgactgatgtttctgtccaacctgtgaaaccgttctctttactgaaccggtcaatctggtcccggctcactgcccaaggggacagatcacacttgttggccaagagcaggcagggcaccggctctccattgggtagtgtgagcttgctgtctaggtcctgtttccacctctggctgttgctgaaggtagtggcattggtaacgtcaaacataataacacaggcagaggcatcccgataatacaatcgtgtcatagaggtgaagcgctcctgccctgcaatatcccacagctgaagccgcactatctcgtagtcagaccactggagaaccttcagagcaaaatccacaaattgtgaggaaggagcagccggcacctcgattccctagacgccctcccgcgcgcctctctctccccttcctccgcaagcgtcacgtgcagggttgcctgtggc

SEQ ID NO: 13749 - RNA, 1346 nt, Homo sapiens
  source 1..1346: mol_type = other RNA
gctgggattacaggcatgagccaccatgcccggccaaaaaacttgactattcttgatgccaagacaagagaaacttaattatgacgttagaagtttcaaaaatacagtgacttctgggacacttctagtagccaaaaatccacagatgcccagaccccctccttctgcattccagaatcagatgtttacattccaagacagaaagaatctgaaacaacggcctacaagaaatttgggaaatgacatttgatctcattttcctctcaattggaagtcatgatatcaatgaatatcaaatggaaaaataagctcagaagtaggtgagaattatgatctctaaaacgcaggtgctgatttctaatccttctcataaaattccggatcacaaattgagggctgatgagaagatcttacaccgaaggcactaactggcactaatgtgagccagcaacatgtgaaaggctaatccaggagatgcagaaatgcacatgggttccaggtgtcttttctaagtgacaatgggcctccttactggacagtagtcaggagacaattcaaatgtacttaataaaattgtcaggtgggcaaccaaagggaagagacttaaaagacctcccagaactgggatggaaaataagccaaacactactagcagcaggaccagctggaggacttggtttgtagattgatgtagtccccttgggtggacaaagacatgatatcttctgtggaatttctcatcatcttttcaatgaggactctcatagcctcattaatatttttgttctccttgactgatgtttctgtccaacctgtgaaaccgttctctttactgaaccggtcaatctggtcccggctcactgcccaaggggacagatcacacttgttggccaagagcaggcagggcaccggctctccattgggtagtgtgagcttgctgtctaggtcctgtttccacctctggctgttgctgaaggtagtggcattggtaacgtcaaacataataacacaggcagaggcatcccgataatacaatcgtgtcatagaggtgaagcgctcctgccctgcaatatcccacagctgaagccgcactatctcgtagtcagaccactggagaaccttcagagcaaaatccacgggacttcccccgagcggctccaagtcagtgactgaatcccagtcagctccttacaccactggggccagatgatggggaccctccccttgcagcacaaaccaaattgtgaggaaggagcagccggcacctcgattccctagacgccctcccgcgcgcctctctctccccttcctccgcaagcgtcacgtgcagggttgcctgtggcact

SEQ ID NO: 13750 - RNA, 1499 nt, Homo sapiens
  source 1..1499: mol_type = other RNA
gctgggattacaggcatgagccaccatgcccggccaaaaaacttgactattcttgatgccaagacaagagaaacttaattatgacgttagaagtttcaaaaatacagtgacttctgggacacttctagtagccaaaaatccacagatgcccagaccccctccttctgcattccagaatcagatgtttacattccaagacagaaagaatctgaaacaacggcctacaagaaatttgggaaatgacatttgatctcattttcctctcaattggaagtcatgatatcaatgaatatcaaatggaaaaataagctcagaagtaggtgagaattatgatctctaaaacgcaggtgctgatttctaatccttctcataaaattccggatcacaaattgagggctgatgagaagatcttacaccgaaggcactaactggcactaatgtgagccagcaacatgtgaaaggctaatccaggagatgcagaaatgcacatgggttccaggtgtcttttctaagtgacaatgggcctccttactggacagtagtcaggagacaattcaaatgtacttaataaaattgtcaggtgggcaaccaaagggaagagacttaaaagacctcccagaactgggatggaaaataagccaaacactactagcagcaggaccagctggaggacttggtttgtagattgatgtagtccccttgggtggacaaagacatgatatcttctgtggaatttctcatcatcttttcaatgaggactctcatagcctcattaatatttttgttctccttgactgatgtttctgtccaacctgtgaaaccgttctctttactgaaccggtcaatctggtcccggctcactgcccaaggggacagatcacacttgttggccaagagcaggcagggcaccggctctccattgggtagtgtgagcttgctgtctaggtcctgtttccacctctggctgttgctgaaggtagtggcattggtaacgtcaaacataataacacaggcagaggcatcccgataatacaatcgtgtcatagaggtgaagcgctcctgccctgcaatatcccacagctgaagccgcactatctcgtagtcagaccactggagaaccttcagagcaaaatccactcccaccgtggacttgtagtgtttgctgaagctgtcctgggaatatcgctgcaccagcgacgtcttgcccactgcggcgtcccccaccaccagcactttgaacaggtggtcgcggctgcccatggctagcggggtgtgcgttttagggaggcgggaagtgtggtcggggatcgggggtcgctcgttttaacccctttggatccggaccctcttcaaactgaagtgaggcattcccacccaccgcctgtctgggcaaattgtgaggaaggagcagccggcacctcgattccctagacgccctcccgcgcgcctctctctccccttcctccgcaagcgtcacgtgcagggttgcctgtggcact

SEQ ID NO: 13751 - RNA, 1600 nt, Homo sapiens
  source 1..1600: mol_type = other RNA
gctgggattacaggcatgagccaccatgcccggccaaaaaacttgactattcttgatgccaagacaagagaaacttaattatgacgttagaagtttcaaaaatacagtgacttctgggacacttctagtagccaaaaatccacagatgcccagaccccctccttctgcattccagaatcagatgtttacattccaagacagaaagaatctgaaacaacggcctacaagaaatttgggaaatgacatttgatctcattttcctctcaattggaagtcatgatatcaatgaatatcaaatggaaaaataagctcagaagtaggtgagaattatgatctctaaaacgcaggtgctgatttctaatccttctcataaaattccggatcacaaattgagggctgatgagaagatcttacaccgaaggcactaactggcactaatgtgagccagcaacatgtgaaaggctaatccaggagatgcagaaatgcacatgggttccaggtgtcttttctaagtgacaatgggcctccttactggacagtagtcaggagacaattcaaatgtacttaataaaattgtcaggtgggcaaccaaagggaagagacttaaaagacctcccagaactgggatggaaaataagccaaacactactagcagcaggaccagctggaggacttggtttgtagattgatgtagtccccttgggtggacaaagacatgatatcttctgtggaatttctcatcatcttttcaatgaggactctcatagcctcattaatatttttgttctccttgactgatgtttctgtccaacctgtgaaaccgttctctttactgaaccggtcaatctggtcccggctcactgcccaaggggacagatcacacttgttggccaagagcaggcagggcaccggctctccattgggtagtgtgagcttgctgtctaggtcctgtttccacctctggctgttgctgaaggtagtggcattggtaacgtcaaacataataacacaggcagaggcatcccgataatacaatcgtgtcatagaggtgaagcgctcctgccctgcaatatcccacagctgaagccgcactatctcgtagtcagaccactggagaaccttcagagcaaaatccactcccaccgtggacttgtagtgtttgctgaagctgtcctgggaatatcgctgcaccagcgacgtcttgcccactgcggcgtcccccaccaccagcactttgaacaggtggtcgcggctgcccatggctagcggggtgtgcgttttagggaggcgggaagtgtggtcggggatcgggggtcgctcgttttaacccctttggatccggaccctcttcaaactgaagtgaggcattcccacccaccgcctgtctgggcgggacttcccccgagcggctccaagtcagtgactgaatcccagtcagctccttacaccactggggccagatgatggggaccctccccttgcagcacaaaccaaattgtgaggaaggagcagccggcacctcgattccctagacgccctcccgcgcgcctctctctccccttcctccgcaagcgtcacgtgcagggttgcctgtggcact

SEQ ID NO: 13752 - RNA, 1476 nt, Homo sapiens
  source 1..1476: mol_type = other RNA
gctgggattacaggcatgagccaccatgcccggccaaaaaacttgactattcttgatgccaagacaagagaaacttaattatgacgttagaagtttcaaaaatacagtgacttctgggacacttctagtagccaaaaatccacagatgcccagaccccctccttctgcattccagaatcagatgtttacattccaagacagaaagaatctgaaacaacggcctacaagaaatttgggaaatgacatttgatctcattttcctctcaattggaagtcatgatatcaatgaatatcaaatggaaaaataagctcagaagtaggtgagaattatgatctctaaaacgcaggtgctgatttctaatccttctcataaaattccggatcacaaattgagggctgatgagaagatcttacaccgaaggcactaactggcactaatgtgagccagcaacatgtgaaaggctaatccaggagatgcagaaatgcacatgggttccaggtgtcttttctaagtgacaatgggcctccttactggacagtagtcaggagacaattcaaatgtacttaataaaattgtcaggtgggcaaccaaagggaagagacttaaaagacctcccagaactgggatggaaaataagccaaacactactagcagcaggaccagctggaggacttggtttgtagattgatgtagtccccttgggtggacaaagacatgatatcttctgtggaatttctcatcatcttttcaatgaggactctcatagcctcattaatatttttgttctccttgactgatgtttctgtccaacctgtgaaaccgttctctttactgaaccggtcaatctggtcccggctcactgcccaaggggacagatcacacttgttggccaagagcaggcagggcaccggctctccattgggtagtgtgagcttgctgtctaggtcctgtttccacctctggctgttgctgaaggtagtggcattggtaacgtcaaacataataacacaggcagaggcatcccgataatacaatcgtgtcatagaggtgaagcgctcctgccctgcaatatcccacagctgaagccgcactatctcgtagtcagaccactggagaaccttcagagcaaaatccactcccaccgtggacttgtagtgtttgctgaagctgtcctgggaatatcgctgcaccagcgacgtcttgcccactgcggcgtcccccaccaccagcactttgaacaggtggtcgcggctgcccatggctagcggggtgtgcgttttagggaggcgggaagtgtggtcggggatcgggggtcgctcgttttaacccctttggatccggaccctcttcaaactgaagtgaggcattcccacccaccgcctgtctgggctcgattccctagacgccctcccgcgcgcctctctctccccttcctccgcaagcgtcacgtgcagggttgcctgtggcactacatt

SEQ ID NO: 13753 - RNA, 1498 nt, Homo sapiens
  source 1..1498: mol_type = other RNA
gctgggattacaggcatgagccaccatgcccggccaaaaaacttgactattcttgatgccaagacaagagaaacttaattatgacgttagaagtttcaaaaatacagtgacttctgggacacttctagtagccaaaaatccacagatgcccagaccccctccttctgcattccagaatcagatgtttacattccaagacagaaagaatctgaaacaacggcctacaagaaatttgggaaatgacatttgatctcattttcctctcaattggaagtcatgatatcaatgaatatcaaatggaaaaataagctcagaagtaggtgagaattatgatctctaaaacgcaggtgctgatttctaatccttctcataaaattccggatcacaaattgagggctgatgagaagatcttacaccgaaggcactaactggcactaatgtgagccagcaacatgtgaaaggctaatccaggagatgcagaaatgcacatgggttccaggtgtcttttctaagtgacaatgggcctccttactggacagtagtcaggagacaattcaaatgtacttaataaaattgtcaggtgggcaaccaaagggaagagacttaaaagacctcccagaactgggatggaaaataagccaaacactactagcagcaggaccagctggaggacttggtttgtagattgatgtagtccccttgggtggacaaagacatgatatcttctgtggaatttctcatcatcttttcaatgaggactctcatagcctcattaatatttttgttctccttgactgatgtttctgtccaacctgtgaaaccgttctctttactgaaccggtcaatctggtcccggctcactgcccaaggggacagatcacacttgttggccaagagcaggcagggcaccggctctccattgggtagtgtgagcttgctgtctaggtcctgtttccacctctggctgttgctgaaggtagtggcattggtaacgtcaaacataataacacaggcagaggcatcccgataatacaatcgtgtcatagaggtgaagcgctcctgccctgcaatatcccacagctgaagccgcactatctcgtagtcagaccactggagaaccttcagagcaaaatccactcccaccgtggacttgtagtgtttgctgaagctgtcctgggaatatcgctgcaccagcgacgtcttgcccactgcggcgtcccccaccaccagcactttgaacaggtggtcgcggctgcccatggctagcggggtgtgcgttttagggaggcgggaagtgtggtcggggatcgggggtcgctcgttttaacccctttggatccggaccctcttcaaactgaagtgaggcattcccacccaccgcctgtctgggctgctcaaattgtgaggaaggagcagccggcacctcgattccctagacgccctcccgcgcgcctctctctccccttcctccgcaagcgtcacgtgcagggttgcctgt

SEQ ID NO: 13754 - RNA, 1551 nt, Homo sapiens
  source 1..1551: mol_type = other RNA
gctgggattacaggcatgagccaccatgcccggccaaaaaacttgactattcttgatgccaagacaagagaaacttaattatgacgttagaagtttcaaaaatacagtgacttctgggacacttctagtagccaaaaatccacagatgcccagaccccctccttctgcattccagaatcagatgtttacattccaagacagaaagaatctgaaacaacggcctacaagaaatttgggaaatgacatttgatctcattttcctctcaattggaagtcatgatatcaatgaatatcaaatggaaaaataagctcagaagtaggtgagaattatgatctctaaaacgcaggtgctgatttctaatccttctcataaaattccggatcacaaattgagggctgatgagaagatcttacaccgaaggcactaactggcactaatgtgagccagcaacatgtgaaaggctaatccaggagatgcagaaatgcacatgggttccaggtgtcttttctaagtgacaatgggcctccttactggacagtagtcaggagacaattcaaatgtacttaataaaattgtcaggtgggcaaccaaagggaagagacttaaaagacctcccagaactgggatggaaaataagccaaacactactagcagcaggaccagctggaggacttggtttgtagattgatgtagtccccttgggtggacaaagacatgatatcttctgtggaatttctcatcatcttttcaatgaggactctcatagcctcattaatatttttgttctccttgactgatgtttctgtccaacctgtgaaaccgttctctttactgaaccggtcaatctggtcccggctcactgcccaaggggacagatcacacttgttggccaagagcaggcagggcaccggctctccattgggtagtgtgagcttgctgtctaggtcctgtttccacctctggctgttgctgaaggtagtggcattggtaacgtcaaacataataacacaggcagaggcatcccgataatacaatcgtgtcatagaggtgaagcgctcctgccctgcaatatcccacagctgaagccgcactatctcgtagtcagaccactggagaaccttcagagcaaaatccactcccaccgtggacttgtagtgtttgctgaagctgtcctgggaatatcgctgcaccagcgacgtcttgcccactgcggcgtcccccaccaccagcactttgaacaggtggtcgcggctgcccatggctagcggggtgtgcgttttagggaggcgggaagtgtggtcggggatcgggggtcgctcgttttaacccctttggatccggaccctcttcaaactgaagtgaggcattcccacccaccgcctgtctgggctgctcgggacttcccccgagcggctccaagtcagtgactgaatcccagtcagctccttacaccactggggccagatgatggggaccctccccttgcagcacaaaccaaattgtgaggaaggagcagccggcacctcgattccctagacgccctcccgcgc

SEQ ID NO: 13755 - RNA, 1201 nt, Homo sapiens
  source 1..1201: mol_type = other RNA
gctgggattacaggcatgagccaccatgcccggccaaaaaacttgactattcttgatgccaagacaagagaaacttaattatgacgttagaagtttcaaaaatacagtgacttctgggacacttctagtagccaaaaatccacagatgcccagaccccctccttctgcattccagaatcagatgtttacattccaagacagaaagaatctgaaacaacggcctacaagaaatttgggaaatgacatttgatctcattttcctctcaattggaagtcatgatatcaatgaatatcaaatggaaaaataagctcagaagtaggtgagaattatgatctctaaaacgcaggtgctgatttctaatccttctcataaaattccggatcacaaattgagggctgatgagaagatcttacaccgaaggcactaactggcactaatgtgagccagcaacatgtgaaaggctaatccaggagatgcagaaatgcacatgggttccaggtgtcttttctaagtgacaatgggcctccttactggacagtagtcaggagacaattcaaatgtacttaataaaattgtcaggtgggcaaccaaagggaagagacttaaaagacctcccagaactgggatggaaaataagccaaacactactagcagcaggaccagctggaggacttggtttgtagattgatgtagtccccttgggtggacaaagacatgatatcttctgtggaatttctcatcatcttttcaatgaggactctcatagcctcattaatatttttgttctccttgactgatgtttctgtccaacctgtgaaaccgttctctttactgaaccggtcaatctggtcccggctcactgcccaaggggacagatcacacttgttggccaagagcaggcagggcaccggctctccattgggtagtgtgagcttgctgtctaggtcctgtttccacctctggctgttgctgaaggtagtggcattggtaacgtcaaacataataacacaggcagaggcatcccgataatacaatcgtgtcatagaggtgaagcgctcctgccctgcaatatcccacagctgaagccgcactatctcgtagtcagaccactggagaaccttcagagcaaaatccactcgattccctagacgccctcccgcgcgcctctctctccccttcctccgcaagcgtcacgtgcag

SEQ ID NO: 13756 - RNA, 1816 nt, Homo sapiens
  source 1..1816: mol_type = other RNA
gctgggattacaggcatgagccaccatgcccggccaataaaggtattttttttaattagtagattaaattattgctgctgagtcagttagcacacctaaatacttgggtaaaccttcttgaaaggctcctaaaacaactgtaaagtaaaagactactgaacagaaacacacaaaataaacagagaaaaatcctggaaaatattgatcctaaagccctcctcagcaatcccctttgtatttgtgaagatttgccgaaaaataatgtacaaattttacaatgaaagtctgccatacttgacaaaataatttcttgtaatagcaggccgaggaattccattccagttttgagactatactcctagtatgtttcacagaagctgtctgaatgccaatttataaaaataataccctatagagtaagtttgtatctatattttaagtgattcagctctaattaccataaagaaaattcaaaaaattttaaatgttatcaaattgaaccatccttcacttctaaattttgaggaaacacatgtaaaaggaagtaaaaattaaatgctgaaatttgaaaaaatctgaattctatatatgttcataagttcatacataaacatttacatctttattacagaataaaagcatactttttgatatgatatactttcagctgtgtgaacatcttcctgatttctcagtactttttgtgtgtccatattgagaacctgaagctgctggatcagctctgcttgctgggctgtatgtgtactgttctgtttgtaaagattctgcagctcctgcagttccttcctgaccagggtaatatccatatccttctggataagttcagtctgtttattactcaactgtaatgatagagcattgtatttactctgtgatacttcaacttctttccttgcttcaattaaattgtcttcaaaggtctttatttttgcatcagtgctatatttttcttttctcaaatgtgcttcctgcttcctcaatttctccaggtcatttagcaggtcagtgcagcgggtacttaatttcttgttttcctcctccagattttttataactagtctgttttgctcttctttgttctgtacacactccttagtgtccttaatttcttgacttttatctttaaatttcttctccaagtcactgaattctttccttaagaaagcattttcttcatctactgcaattttccgttttacaaggtcatttatttcctgtttcagtactgactctctctgttcaaattcttgtattttggcatccttgacttgcagaatttctagaacttttctgtctttagcttcagatttctgtttttctctttccacaaccaaactgaccacttgtgtgagatctgggtttgtaacctggagacgtttccacaaagaccatacaaattctttatcagcctgacacagggccaactcctcctttaggctgctcagctcttcctccagcagctgcgtccgggtcaccatcgcctcctctaccgagatgccctctagccgtctggaccccatgggcgcgctgaggaggggagcatgagccggagctgcccccccaggccctcgccggccccctgacccttcttcacccacccagattttatcactttcgtccgcgaccacctcccgcgctgcgccggcaaaacccgaggcctcgctgcgcattgcgtgtacttcagctccccgcccaacacgtggggacctggggcccagctgtcgcgctgggggcgaagggtgcggtgagggaggcgaacgcgccgccatggctgcggctgctaacgggtcaagtt

SEQ ID NO: 13757 - RNA, 1609 nt, Homo sapiens
  source 1..1609: mol_type = other RNA
gctgggattacaggcatgagccaccatgcccggccaatgccatctattaaaaaaacaaagaaaaagagtacacaaccacaaagcactgggccaaatgcattgtttccatgtttgcaaggatttaccatagaaatattaggttgatgcaaaaattaaatttccagactgcgaattttaaatcattgtaactacgctaaaacatattctattaatcaaaacaggaaccattacaatcaacacatttttgccaatgagaaatgtttgtttattcctgtagcataaaaatccgtgcttcaggatttgacgaactcttggaaagcattttctgcaccatgctgaagtgttttccctgcaaaaagttgtcaagatgctagcagaagtggtagtcagttggcgaaaggtcaggtgaatatggtggatgaggcaaaactttgtagcccaattccttcaacttttgaagcactggttgtgcgacacgcagtcaggtgttgtcgtggagaagaattgggccctttctgttgaccaatgcaggcagcaggtattgcagttttcggtgcatcttaccaatttgctgagcatacttctcagatgtaatggtttcaccaggattcagaaaactgtagtggatcagatgggcagcagaccaccgaacagtgaccatgaccttttttttggtgcaagtttggctttgggaactgctttggagctgcctcttggtccaaccactgagctggttgttgtataaaattcacttttcattacatgtcacaatccgattgagaaatggtttgttgttgcgtagcataaaagaagactacacttcaaaacgatagttttgatttccgctcagctcatgaggcacccacttatcaagctttttcacctttccaatttgcttcgaatgctgaacgaccctaatgaccgtagaatagtcaacgctgagttcttctgtaatttttcatgtagttcaatgattgctctcaattggtcgttgtcaacttcccatggcccatatcacgttcctcatcttcaaggctctcttccttgcaaaacttcttaagccaccactgcactgtatgtttgttagcagttcctgggccaaatgtgttactgatgttttgagttgtcttcgctgctttatgaaccattttgaactcgaataagaaaactgctccaaatttgctttttatctaacatcattagacaaaaagcatattagacgctctgctgagcggctgggagaatccgtcgcgccagtcagggcccggcttcttccaacaacagacactttgcgagccttccagaagccttggctaagcgagaaggcagggtggaggccgccactgcgaggacggtccccacccagctgcgaggagctcgcggttccccagaggggcgggcctgcgtccgggtaaccgtgcgcgacgtccacgagtttttaggacgaccagcccttcagcctctaggccccgacgcctgcgccatttaagccacatatccgcccgcccggccgcggccaaggccggcggcagctacgtagccgccgccgcccggggccccacagcccacgggccggatggaccgagcgccggctgcggcgttccggtgc

SEQ ID NO: 13758 - RNA, 1636 nt, Homo sapiens
  source 1..1636: mol_type = other RNA
gctgggattacaggcatgagccaccatgcccggccaatgccatctattaaaaaaacaaagaaaaagagtacacaaccacaaagcactgggccaaatgcattgtttccatgtttgcaaggatttaccatagaaatattaggttgatgcaaaaattaaatttccagactgcgaattttaaatcattgtaactacgctaaaacatattctattaatcaaaacaggaaccattacaatcaacacatttttgccaatgagaaatgtttgtttattcctgtagcataaaaatccgtgcttcaggatttgacgaactcttggaaagcattttctgcaccatgctgaagtgttttccctgcaaaaagttgtcaagatgctagcagaagtggtagtcagttggcgaaaggtcaggtgaatatggtggatgaggcaaaactttgtagcccaattccttcaacttttgaagcactggttgtgcgacacgcagtcaggtgttgtcgtggagaagaattgggccctttctgttgaccaatgcaggcagcaggtattgcagttttcggtgcatcttaccaatttgctgagcatacttctcagatgtaatggtttcaccaggattcagaaaactgtagtggatcagatgggcagcagaccaccgaacagtgaccatgaccttttttttggtgcaagtttggctttgggaactgctttggagctgcctcttggtccaaccactgagctggttgttgtataaaattcacttttcattacatgtcacaatccgattgagaaatggtttgttgttgcgtagcataaaagaagactacacttcaaaacgatagttttgatttccgctcagctcatgaggcacccacttatcaagctttttcacctttccaatttgcttcgaatgctgaacgaccctaatgaccgtagaatagtcaacgctgagttcttctgtaatttttcatgtagttcaatgattgctctcaattggtcgttgtcaacttcccatggcccatatcacgttcctcatcttcaaggctctcttccttgcaaaacttcttaagccaccactgcactgtatgtttgttagcagttcctgggccaaatgtgttactgatgttttgagttgtcttcgctgctttatgaaccattttgaactcgaataagaaaactgctccaaatttgctttttatctaacatcattagacaaaaagcatattccaatacaacccccacttccgacctacagacgctctgctgagcggctgggagaatccgtcgcgccagtcagggcccggcttcttccaacaacagacactttgcgagccttccagaagccttggctaagcgagaaggcagggtggaggccgccactgcgaggacggtccccacccagctgcgaggagctcgcggttccccagaggggcgggcctgcgtccgggtaaccgtgcgcgacgtccacgagtttttaggacgaccagcccttcagcctctaggccccgacgcctgcgccatttaagccacatatccgcccgcccggccgcggccaaggccggcggcagctacgtagccgccgccgcccggggccccacagcccacgggccggatggaccgagcgccggctgcggcgttccggtgc

SEQ ID NO: 13759 - RNA, 1613 nt, Homo sapiens
  source 1..1613: mol_type = other RNA
gctgggattacaggcatgagccaccatgcccggccaatgccatctattaaaaaaacaaagaaaaagagtacacaaccacaaagcactgggccaaatgcattgtttccatgtttgcaaggatttaccatagaaatattaggttgatgcaaaaattaaatttccagactgcgaattttaaatcattgtaactacgctaaaacatattctattaatcaaaacaggaaccattacaatcaacacatttttgccaatgagaaatgtttgtttattcctgtagcataaaaatccgtgcttcaggatttgacgaactcttggaaagcattttctgcaccatgctgaagtgttttccctgcaaaaagttgtcaagatgctagcagaagtggtagtcagttggcgaaaggtcaggtgaatatggtggatgaggcaaaactttgtagcccaattccttcaacttttgaagcactggttgtgcgacacgcagtcaggtgttgtcgtggagaagaattgggccctttctgttgaccaatgcaggcagcaggtattgcagttttcggtgcatcttaccaatttgctgagcatacttctcagatgtaatggtttcaccaggattcagaaaactgtagtggatcagatgggcagcagaccaccgaacagtgaccatgaccttttttttggtgcaagtttggctttgggaactgctttggagctgcctcttggtccaaccactgagctggttgttgtataaaattcacttttcattacatgtcacaatccgattgagaaatggtttgttgttgcgtagcataaaagaagactacacttcaaaacgatagttttgatttccgctcagctcatgaggcacccacttatcaagctttttcacctttccaatttgcttcgaatgctgaacgaccctaatgaccgtagaatagtcaacgctgagttcttctgtaatttttcatgtagttcaatgattgctctcaattggtcgttgtcaacttcccatggcccatatcacgttcctcatcttcaaggctctcttccttgcaaaacttcttaagccaccactgcactgtatgtttgttagcagttcctgggccaaatgtgttactgatgttttgagttgtcttcgctgctttatgaaccattttgaactcgaataagaaaactgctccaaatttgctttttatctaacatcattagacaaaaagcatattctacagacgctctgctgagcggctgggagaatccgtcgcgccagtcagggcccggcttcttccaacaacagacactttgcgagccttccagaagccttggctaagcgagaaggcagggtggaggccgccactgcgaggacggtccccacccagctgcgaggagctcgcggttccccagaggggcgggcctgcgtccgggtaaccgtgcgcgacgtccacgagtttttaggacgaccagcccttcagcctctaggccccgacgcctgcgccatttaagccacatatccgcccgcccggccgcggccaaggccggcggcagctacgtagccgccgccgcccggggccccacagcccacgggccggatggaccgagcgccggctgcggcgttccggtgc

SEQ ID NO: 13760 - RNA, 1372 nt, Homo sapiens
  source 1..1372: mol_type = other RNA
gctgggattacaggcatgagccaccatgcccggccaatgccatctattaaaaaaacaaagaaaaagagtacacaaccacaaagcactgggccaaatgcattgtttccatgtttgcaaggatttaccatagaaatattaggttgatgcaaaaattaaatttccagactgcgaattttaaatcattgtaactacgctaaaacatattctattaatcaaaacaggaaccattacaatcaacacatttttgccaatgagaaatgtttgtttattcctgtagcataaaaatccgtgcttcaggatttgacgaactcttggaaagcattttctgcaccatgctgaagtgttttccctgcaaaaagttgtcaagatgctagcagaagtggtagtcagttggcgaaaggtcaggtgaatatggtggatgaggcaaaactttgtagcccaattccttcaacttttgaagcactggttgtgcgacacgcagtcaggtgttgtcgtggagaagaattgggccctttctgttgaccaatgcaggcagcaggtattgcagttttcggtgcatcttaccaatttgctgagcatacttctcagatgtaatggtttcaccaggattcagaaaactgtagtggatcagatgggcagcagaccaccgaacagtgaccatgaccttttttttggtgcaagtttggctttgggaactgctttggagctgcctcttggtccaaccactgagctggttgttgtataaaattcacttttcattacatgtcacaatccgattgagaaatggtttgttgttgcgtagcataaaagaagactacacttcaaaacgatagttttgatttccgctcagctcatgaggcacccacttatcaagctttttcacctttccaatttgcttcgaatgctgaacgaccctaatgaccgtagaatagtcaacgctgagttcttctgtaatttttcatgtagttcaatgattgctctcaattggtcgttgtcaacttcccatggcccatatcacgttcctcatcttcaaggctctcttccttgcaaaacttcttaagccaccactgcactgtatgtttgttagcagttcctgggccaaatgtgttactgatgttttgagttgtcttcgctgctttatgaaccattttgaactcgaataagaaaactgctccaaatttgctttttatctaacatcattagacaaaaagcatattctcggcgtctcgtctctcgcccgctgccccgcgagcccgcggcccccgggctcccgccatccgccgacaccgggagcccgggctccccgcgccctgccctccgcgccgggggccgcccgccgcagacacgggacccgcttcgaggccgctttggc

SEQ ID NO: 13761 - RNA, 1646 nt, Homo sapiens
  source 1..1646: mol_type = other RNA
gctgggattacaggcatgagccaccatgcccggccaatgccatctattaaaaaaacaaagaaaaagagtacacaaccacaaagcactgggccaaatgcattgtttccatgtttgcaaggatttaccatagaaatattaggttgatgcaaaaattaaatttccagactgcgaattttaaatcattgtaactacgctaaaacatattctattaatcaaaacaggaaccattacaatcaacacatttttgccaatgagaaatgtttgtttattcctgtagcataaaaatccgtgcttcaggatttgacgaactcttggaaagcattttctgcaccatgctgaagtgttttccctgcaaaaagttgtcaagatgctagcagaagtggtagtcagttggcgaaaggtcaggtgaatatggtggatgaggcaaaactttgtagcccaattccttcaacttttgaagcactggttgtgcgacacgcagtcaggtgttgtcgtggagaagaattgggccctttctgttgaccaatgcaggcagcaggtattgcagttttcggtgcatcttaccaatttgctgagcatacttctcagatgtaatggtttcaccaggattcagaaaactgtagtggatcagatgggcagcagaccaccgaacagtgaccatgaccttttttttggtgcaagtttggctttgggaactgctttggagctgcctcttggtccaaccactgagctggttgttgtataaaattcacttttcattacatgtcacaatccgattgagaaatggtttgttgttgcgtagcataaaagaagactacacttcaaaacgatagttttgatttccgctcagctcatgaggcacccacttatcaagctttttcacctttccaatttgcttcgaatgctgaacgaccctaatgaccgtagaatagtcaacgctgagttcttctgtaatttttcatgtagttcaatgattgctctcaattggtcgttgtcaacttcccatggcccatatcacgttcctcatcttcaaggctctcttccttgcaaaacttcttaagccaccactgcactgtatgtttgttagcagttcctgggccaaatgtgttactgatgttttgagttgtcttcgctgctttatgaaccattttgaactcgaataagaaaactgctccaaatttgctttttatctaacatcattagacaaaaagcatattctttgccacggggtggcggcggcggcgcccggcgctttgcatagtgggccgggccgctcccctcccctccccgcccgcggccgggcgaagcgagcgggttccccctgaccggcccggccggcgcaagggtgggggtggagggggaatggccgcggccccgccttatagttggccctccgccagcgccgccattttgttctcgacggagatggctccggctgggcgggctcccttcctccttatcctcctcctcctcccgcctgcagtcccttcttccttctctgccgggattttcacccctccgcttctagtccgcctttggcggccgtcgcagcccaaccgccgttttttctgaaggggagggtaaaagaaaaggaggaaggcgggtgcgaggcgcgacctcgtgagcgacggatgggctggctaatt

SEQ ID NO: 13762 - RNA, 2470 nt, Homo sapiens
  source 1..2470: mol_type = other RNA
gctgggattacaggcatgagccaccatgcccggcccagagttaagtctcttattgggctcctggtttgcactcttgggcccacaagagttattctctatacagccaccagaaaaaaaaagaaagaaagaaagaaactaagtactcatctaaaaattatctaaaaaagaacaatgaaagaaaccagaagaaactaggaaaaaattaagaagaatgaagtaaaaattaattaactagggaataaaaattgtagtaagtagaataagtaaaaaagcttatactttgaaaatacctatagataaaacatttgcaagactgatcacaaaaaaagcaaacattgacaagattactatccagaaataagacataaactctgatataatacatactgatagaattctaggacaataaatagagcatgcaggtgtgtgacagcagatttgaaaacacagaggtactaaatggtttccatttagtatatggtgaccaaaattgaccaaagtagaagtggaaaactgaaaagaccaatttcagagatgaaattagaagagttatttgacgtttaatggcaaaaaccaccagggaagtttggataaactattacaaatatcctctcaaaaccattataagagatcaagagaaagtaagggaaattcccagggaaccaaatagaggtgaaaacaggaggagtaagctacagctgggaccgaagctctgaagtccagcttgccaacctcagtaacaaaggagtttagaatacagtgactgtggcaggacaagacatagtcccatgggactacataaagtagggagaggaactgagaccctgacatgaagctggggcaccagaaatgaaaaggtaaatcagaaaaaaaaaaaaaaaaaaaaatcttccaagaaagctcaggtgtttcagcaagggctctaggtgggctctgtgtgtttcttccctatcacattctcaagtcattccctcaagataactattatcctggattttgtgtttgtgtttacacagagttctgcttgattttaagtaaaaaattgtatactaaggtagtcttctgtgacttgagtttttcacttagtattgtgtttatgaaaaaatttaaaccctatgtttactgataaccacaaggaataacagacacaatatttaataaaaaaaggaacaaaatatcgaaaccatctatatactgtaatgtacctttaaaccaatgctagggaaaaacaaagggaaaacacaaaactgcaataaacttcatcttctctcccaggtttttcttgaacaattcccacccccattccctactatgtatccttaacttctttagacagtgaatgagaaattaatactaaaagccctcaaatgaaccctagggacatttcctgggttttcccttcttctcccctctccaaccgtgccgtgaagggcaagcccctcagccctaaaatctgaggaggcccagagtggtggctggggcagaggagtgggctacccctgcagagtagagacgtgtatagtgggggatatccactgggagccccagtcccaggtgaaagcacactggtgctcctgggcaaggaggcccggctgtccccacaatctcccgtggggaagcatcattggttggtcgactgcccatcttgctgcggttatagaaccaaactcgaaccacatccttctgcagctggaggcacccagcaatgtggctgatttgctggggtgtgggcttagggcaccgctggaagaatttctccaggctgtttccgattcgtcgctctctgcttgcccgtctccacttcccagactgttgcaggatcatctccattttgcataagcccagaaggttctctgcttccacttccttcagccactttttcagcagtggtcgcagcttccacatgttggcgacgcttagctgctgggcctcgaagcggcagatggtcgtctggctaagcaccttcccaaacagagctcccacagcgatccccacatcggcctgcgagtaccctaggctcaacctcttctgcctcaactccttggccaattgctgcaactctttcagtatgcccgagatgtcctctggcggcggcaacttcggaatgctccgcagggcaatgtagggccccgggagggcgccttcggaggggcgtcgcaaccagtcccctgcctcactagctccaagacggggcctgcagggtgctatccagccccggaattcgtgtggcaggggacccaggggaatcctccacacgtcagggcctgggcagatccctggcctgactgccggccagaccatcaccctgccaggggccgcctgggtgctcaaccaggtcagagtgtcaacccgcaggggcatcggccctctggggccgcccccaccactgcctggaagggggcagaagtggtttgagggcctgtgtccggccatgggtggaatggcacccgcagcggctctggtaggaact

SEQ ID NO: 13763 - RNA, 7994 nt, Homo sapiens
  source 1..7994: mol_type = other RNA
gctgggattacaggcatgagccaccatgcccggccctggccagtaattcttaaatgagaacttcaagttataaatgtcccttcacttacatttcttttcatcttaacagtgaatgcctcgatagctacattctttttgctgtgcacatttcgagatttaggtatcactaaataagtttggtgttccctgtttttttgtgtgtgtgtgtgatggagtcttgctctgtcacccaggctggagtgcagtggtgtgatctcagctcactgcaacatcggcttcctgggttcaagcgattctcctgcctcagcctccggagtagctgggactacacacgtgccaccaagcccggctaatttttgcatttttagtagagatggggtttcaccatattggccaggctggtctcgaactcctgaccttgtgatctgcctgccttagcctcccaaagtgttatgattacaggtgtgagccaccgcgcccagcgcctgatttatttatttttttgagacagagcctcgctctatcacccaggctggagtgcagtggtgtgatcttggctcactgcaagctccacctcccaggttcacgccattctcctgcctcagcctcctgagtagctgggactacaggcgctggccacctcacctggctaattttttgtatttttagtagagacggggtttcaccgtgttagccaggatggtctcgatctcctgacctcgtgatccacccgccttggcctcccaaagtgctgggattacaggcgtgagccaccgcgcctggcctggtttatttaatgttagcattctgacaagatgttaaatgacccggatacaatgagtaataattgtgttctaagttgcaaagatcccataagggaaataaagaattattaaatatcatcaccaacttcacagatttggtctcaaagtaaatctgctacatactaaataatttaaattaatatggtgatggagtgtgtggcgttggaagaaaacttgttgaagaaagcttactttatttttattcatttaagaggcaaggtttcactctgtcactcaggctggaatgcagtggccccatcatggctcactgcagccttgaactcctgggctcaagtgacccttctgcctcagcttcccaagtagctgggattacagacatgcaccatcatggctaactttttttttgagatggagttttgttcttgttgcccagactggagtgcaatgccgtgatctcggctcactgcaacctcctcctcccaggtacaagtgattctcttgtctcagcctcccaagtagctcggattacaggcatgtgccaccatgcccggctaatttttttgtatttagtagagacggggtttcaccatgttattcaggctggtcgcgaactcctgaactcaggtgatccacccacctcggcctcccaaagtgctgggattacaggcttgcgtcactgcacccagcctctcatggctaattaaattttttttttgtagagatgagtcttgctatgttgtccagctggtctcaaacgcctgggctcaagcggtcctcccaatttggcctccccaagcactgggattacaggtgtgagacaccacccccagttgaaaagttactttggatataactgatttgaattttattcttgtgaaatagtgatgagattttatattgtctacttctaagcggcagacagtcatcatgaggcaaataaaattttctaaggtaaggagagtgagaatggcctttcccctttagtctatggcaaaataaaggggggcatgggagaatcctgatggtggaaatcattttattctcatacacaggttattacagcacaattaggaagagacaatcacaactcacacaatgctatattcaaattatgccaaagtcccaacatattcatttcatttgcaagttaattcctaaaagatcagagcagagtgatacacaagtttattaacacagactacaacgtcaatgaagcctcctggcattgtcggaaatagaaaacatgtataaaaatcttcgaaatgcaggttaaaatgcaaatccaagtgaaaggaaaaagcactactgtgaagcctaacggcaattatttcccttcaaaggaggtttgtgtccagctggagagaaggcctggtggacagaagacaaaggaaggcaaaattcctaagggagaaattcaaaaaaatgatgggggtgctgccctctgctgggcctctttggcagtcgacttcaacttaatgcattagcgccgtaaggttgtaagagaagcaactctggcttgatcttagaaaagctgattttctttttggcagcatatttccggtgagaactgatgggaaaggtggtgtggattcgtggacgaagtctctaacgtaatcttgactactgaagggtaaagacttgcccacaggttagagattacatgaattatccacaacgaatggtagcagatgatgggtcaggggtattttaattgtacagcataacactttagagagctgggaagtatgggacatcattcccgtctttcttcactcagtaactgattatcttgtttcttgtccacagatatttaacctaaataacaatgctttttgaaggttgtttggctaacccagaggtagtaaaagacttcataagtctttctattactgaagaggagcttagtaataactgcaagtctatttatatatgtagcagatggtaacaatctccagagccactgacatatgcagcagaaaagcacaaagaactttgtatttgttataatttctactgcattgtccagatacagatagaaaatactgatatgtagtgtggggaatcttgagacatttcagcctatgcactatgcggcacttgtactgataactgattatcacaattttattaaatgctcatcatttaacagatggcacagaaaataaatggcacactcagaatattaactcaagaacaattaataaaggcactatttacaaatatgtgttcacaattaaagacacccaaccagtgggttggggaagcacccagtagtagttaagtctgaagatcatggagagggaatggtgtcaactgaaaccgagagatctacagccatagatggggcttcccaaaggaagctgtatccttacgggaacacagaagctaccatggtccaggcaggaggaagggaacggtaataaataactttttctcctcccacctctggtatctcccactgttcaaacctatgaagaaaccccagtctctagaagacagcctcaggggggagcagagcagaaaatgggggaaaagggatcaaagaaatagggaatactcagcacacatgcagatccacaatacatacaatttctgtcatgtgcctgctacaaattcaagctaccccgagccctgaaggaataggcttctaactcagatgatgcagtctactcaactatatttaaaaattcacacttaagtgttatcgtcatcacactttacttctaaataaactccaaatacgttatcattactttggctttaagcagccaattcccttttaaaaagattttaaaaagagagaaatatcttttatatttacccacatattcaccattttcagaacttcattcctttgtacagacccaaacttaagttttgtattattttcctgctgccctcaaacatcctttaatgtttcccaaagacaggtctacaggtaataaaattacctttgatttagtttctcagaaacagtctttattttgccttcatttttgaaaacgtttttgacagtaacagaattctaggttgcagggtttgttgtttatttcattaaggaatttagagataatactccattgtcttatagcttgcatagttctcaccagaaatatgctgccattctttgttcatgtgtatgtattatctttttttctcaaggtgttttaaaagtattctgtttatcagtgcttttcatgaatgtgactctgaggtgcactgctgtgatgtaaattatgtttattctacttcaggtcatttgagcttcttgaatatgtgggggtattgttttcaccagatttggaaaatctttagccattatttattcaaatacttcttcatgcctcttcattttctcctctccttctgggactccagttaaacatatattacactactgtaatggttttcctattctcttcctcttctctaagtctttttttctctctgtatatcactttggtagtttttattcttactcttcaagttcattgattttttcttctttttctgtatctaatctctccactcgggattttaacaaaatcagaagttgatttcatccctagaagttccattttggccagtaaaaatatctcttatacctcaggtttcatcaatcttatgttttcctctactttatatttacaatagctcttttaatatccttgtctactaattccatcacctctgtcttttctgggtttctactgatttttctcctggttataagtcatattttattgcttctttgcataacacattagtttttttggatgccggacactgtaggtccagagtagcttttaatctagagttaattagctgcactactaaaacaaaacctttctgagaattctacctgatgctccatgtgtttccactctgtttccactctggctgctgagaacataaactattcccagccctgcatgagttccaggaattgttcagcctgctgctttccagtgcttcttttcctggcctcagtgcaagtcagtactaagtcaaaggactcaggggactcccagcagacttcttgagccctgtatctagaaggatcccatctctccagtactttcccctggaaattctagctgctgtggcctccccaactgccagtcctgtctcttcaattcagcgagatttattgtttcccttccctgaactgcaacctaggaactgccatgcgggggcaggctgagaaaccatggtgctcacctcactctgtctgcagtctcctgaggatcacaaacctgtgcttgtcctatgtctaaaaaccattacctattatacgtattgtatagcttccagttgtttaaggcaggagaggaaatctgacccttgttattccatcacagcagtaaggagaactcttcacatctaagtaaacacacctcacacttacaattcactgctttttgtaataattgatgtataaagaacaccacttccttacagaactatttcaatagcatcatgcttgtcaaattctttacattattgagactactcttcagtatgaacctctgtaggtattattctcaagtgtacagtgagttgtcctttcttgaaatcttccactttgttataaaaaacaatagaattttcttcctgtttaggtattctaaacatttaataaactgacttttgactaaaagcttctctactatcacaacactaataaggttttcacctcaatgagtcatccaatatgtaacgagtagtgtcttctgggagatgactttttttacactgtttgctttttaaaaacttctctttctaaattctgcttagtgactcttgactcctcaattcaagctttttcaacagtcactgcctcaatagggtttctctcccacatgcatcctcaaaagtgtcagaaagtatgacacttgatagcaacctttctgcattcgccaaagtcatgatttttatattatatgatttctctgatgtatcataagctgcgacttcctgttgaaggtggtcccacactcattgcatccatagtatttatctcctgtatgaatcctctgatgcctcataaggtgtgactttcttgtgaaagatttcccacattcaccacatttatatggtctctctcctgtatgaattctctgatgtataatcagctgtgccttctcaaagaaagcttttgcacaatcgctgcatccataggttttctctcctgtgtgatttctttgatgcttaatgagctgcactttctgaacaaatgctttcccacattcactgcattcatagggtttctcccctgtatgaattctctgatgcctaagaagctgtggcttccaggcaaaagctttcctacattcactacattcaaagggcttttctccagtatgggttctctgatgatgaatgagacttgacttctcactgaaggttttcctgcattcactgcattcatagggtttctcacctgtatgtgttctctgatgtgatatcaggcttgacttctgggtgaaggccttcccacactcactgcattcataaggcttctccccagtgtgtgttctgtgatgcgttaggagctgggacttcccaaagaaggttttcccacattgaatgcatccatatggtttctctcctaagtgaattttttgatgtcttattaactctgacttcttaaagaaggcctcctcacaatcactgcatcgatagttcttctctcctgtgtgagttatctgatgtttaatcagctgtggttttctgatgaaggcttcaccacattcgttgcattcgtagggcttctctcctgtatgaatcctctgatgcctaatgagaagtgagttcctgctgaaggctttttgacactcaccacatccgtaaggtttcttccctgtgtgggtcctctgatgagtaatcagctgcgacttccaaaagaaggcttttccacagtgactacatggatagggtttctctcctgtgtgcgctctctgatgtgtgatgagttttaatttctgggagaatgctttcccacactcactgcaactgtagggtttctctattgtgtgcgttatctgatgtcttttaagctgcgacttcctactgaaggcttttccacattcactgcatccatacggcttctctccagtatgaattctctgatgtaaaatgaggagtgacttcctactaaaagctttctgacattcgctgcacccatgcggtttttctcctgagtgagttctttgatgaaccgtgagcagtgacttctgtgaaaaggcttttccacactcactgcattgatagggcttctctcctgtatgagttctctggtgtataacaagttgtgacttcttgttaaaaaatctgccacattccatgcataaatagactcctgtgtgtgttatgtgattagcagtgagccatggctcttcgttgctggattttctacatgtactgcaatcacagtattttatcccaccatgggttctgccaggtttgatacagaacaataatttcttattgagttcatcaattttctttctttcacaattattttttggaataagcaaatcaaaaggacatttcaaacttttttctcctgtgccacatttatgggatcgcagtcctacatgaacaatgtttatgcttgaattaaatatttttccaaaaacatcatatttatggcctctctccatacttttaaggttgtcttgattatctcggagccacattttgggattatctagccagacttccaagaaaaccagattgctatagttctccaacatcacatctctgtacaagttcttctgagtaggattaagtagctgccattcctccagcgtgaaatccacagccacatcctcaaatgatatctgtgactggatcattttccgctgctcttgggaaatctgctgttttgtgacttctcttagtcctgacaccctggagtggcctctggtcagtggtctgtaaactgagaatacatccttggtcttgtgggctcttctttcttatctcacatgaattgtcttgttccagagggctattgcactttacatttcttcactgcccatggaccaggccacttagatgaagccagacacggaatcagagccaaagaactgaaggacacgcagctgcacagggacgctctttccttcatcagaatgagtccctcggacctcgcagggccgcggcggacacggcccgatcggggacgtgaacgcgcagaactac

SEQ ID NO: 13764 - RNA, 7964 nt, Homo sapiens
  source 1..7964: mol_type = other RNA
gctgggattacaggcatgagccaccatgcccggccctggccagtaattcttaaatgagaacttcaagttataaatgtcccttcacttacatttcttttcatcttaacagtgaatgcctcgatagctacattctttttgctgtgcacatttcgagatttaggtatcactaaataagtttggtgttccctgtttttttgtgtgtgtgtgtgatggagtcttgctctgtcacccaggctggagtgcagtggtgtgatctcagctcactgcaacatcggcttcctgggttcaagcgattctcctgcctcagcctccggagtagctgggactacacacgtgccaccaagcccggctaatttttgcatttttagtagagatggggtttcaccatattggccaggctggtctcgaactcctgaccttgtgatctgcctgccttagcctcccaaagtgttatgattacaggtgtgagccaccgcgcccagcgcctgatttatttatttttttgagacagagcctcgctctatcacccaggctggagtgcagtggtgtgatcttggctcactgcaagctccacctcccaggttcacgccattctcctgcctcagcctcctgagtagctgggactacaggcgctggccacctcacctggctaattttttgtatttttagtagagacggggtttcaccgtgttagccaggatggtctcgatctcctgacctcgtgatccacccgccttggcctcccaaagtgctgggattacaggcgtgagccaccgcgcctggcctggtttatttaatgttagcattctgacaagatgttaaatgacccggatacaatgagtaataattgtgttctaagttgcaaagatcccataagggaaataaagaattattaaatatcatcaccaacttcacagatttggtctcaaagtaaatctgctacatactaaataatttaaattaatatggtgatggagtgtgtggcgttggaagaaaacttgttgaagaaagcttactttatttttattcatttaagaggcaaggtttcactctgtcactcaggctggaatgcagtggccccatcatggctcactgcagccttgaactcctgggctcaagtgacccttctgcctcagcttcccaagtagctgggattacagacatgcaccatcatggctaactttttttttgagatggagttttgttcttgttgcccagactggagtgcaatgccgtgatctcggctcactgcaacctcctcctcccaggtacaagtgattctcttgtctcagcctcccaagtagctcggattacaggcatgtgccaccatgcccggctaatttttttgtatttagtagagacggggtttcaccatgttattcaggctggtcgcgaactcctgaactcaggtgatccacccacctcggcctcccaaagtgctgggattacaggcttgcgtcactgcacccagcctctcatggctaattaaattttttttttgtagagatgagtcttgctatgttgtccagctggtctcaaacgcctgggctcaagcggtcctcccaatttggcctccccaagcactgggattacaggtgtgagacaccacccccagttgaaaagttactttggatataactgatttgaattttattcttgtgaaatagtgatgagattttatattgtctacttctaagcggcagacagtcatcatgaggcaaataaaattttctaaggtaaggagagtgagaatggcctttcccctttagtctatggcaaaataaaggggggcatgggagaatcctgatggtggaaatcattttattctcatacacaggttattacagcacaattaggaagagacaatcacaactcacacaatgctatattcaaattatgccaaagtcccaacatattcatttcatttgcaagttaattcctaaaagatcagagcagagtgatacacaagtttattaacacagactacaacgtcaatgaagcctcctggcattgtcggaaatagaaaacatgtataaaaatcttcgaaatgcaggttaaaatgcaaatccaagtgaaaggaaaaagcactactgtgaagcctaacggcaattatttcccttcaaaggaggtttgtgtccagctggagagaaggcctggtggacagaagacaaaggaaggcaaaattcctaagggagaaattcaaaaaaatgatgggggtgctgccctctgctgggcctctttggcagtcgacttcaacttaatgcattagcgccgtaaggttgtaagagaagcaactctggcttgatcttagaaaagctgattttctttttggcagcatatttccggtgagaactgatgggaaaggtggtgtggattcgtggacgaagtctctaacgtaatcttgactactgaagggtaaagacttgcccacaggttagagattacatgaattatccacaacgaatggtagcagatgatgggtcaggggtattttaattgtacagcataacactttagagagctgggaagtatgggacatcattcccgtctttcttcactcagtaactgattatcttgtttcttgtccacagatatttaacctaaataacaatgctttttgaaggttgtttggctaacccagaggtagtaaaagacttcataagtctttctattactgaagaggagcttagtaataactgcaagtctatttatatatgtagcagatggtaacaatctccagagccactgacatatgcagcagaaaagcacaaagaactttgtatttgttataatttctactgcattgtccagatacagatagaaaatactgatatgtagtgtggggaatcttgagacatttcagcctatgcactatgcggcacttgtactgataactgattatcacaattttattaaatgctcatcatttaacagatggcacagaaaataaatggcacactcagaatattaactcaagaacaattaataaaggcactatttacaaatatgtgttcacaattaaagacacccaaccagtgggttggggaagcacccagtagtagttaagtctgaagatcatggagagggaatggtgtcaactgaaaccgagagatctacagccatagatggggcttcccaaaggaagctgtatccttacgggaacacagaagctaccatggtccaggcaggaggaagggaacggtaataaataactttttctcctcccacctctggtatctcccactgttcaaacctatgaagaaaccccagtctctagaagacagcctcaggggggagcagagcagaaaatgggggaaaagggatcaaagaaatagggaatactcagcacacatgcagatccacaatacatacaatttctgtcatgtgcctgctacaaattcaagctaccccgagccctgaaggaataggcttctaactcagatgatgcagtctactcaactatatttaaaaattcacacttaagtgttatcgtcatcacactttacttctaaataaactccaaatacgttatcattactttggctttaagcagccaattcccttttaaaaagattttaaaaagagagaaatatcttttatatttacccacatattcaccattttcagaacttcattcctttgtacagacccaaacttaagttttgtattattttcctgctgccctcaaacatcctttaatgtttcccaaagacaggtctacaggtaataaaattacctttgatttagtttctcagaaacagtctttattttgccttcatttttgaaaacgtttttgacagtaacagaattctaggttgcagggtttgttgtttatttcattaaggaatttagagataatactccattgtcttatagcttgcatagttctcaccagaaatatgctgccattctttgttcatgtgtatgtattatctttttttctcaaggtgttttaaaagtattctgtttatcagtgcttttcatgaatgtgactctgaggtgcactgctgtgatgtaaattatgtttattctacttcaggtcatttgagcttcttgaatatgtgggggtattgttttcaccagatttggaaaatctttagccattatttattcaaatacttcttcatgcctcttcattttctcctctccttctgggactccagttaaacatatattacactactgtaatggttttcctattctcttcctcttctctaagtctttttttctctctgtatatcactttggtagtttttattcttactcttcaagttcattgattttttcttctttttctgtatctaatctctccactcgggattttaacaaaatcagaagttgatttcatccctagaagttccattttggccagtaaaaatatctcttatacctcaggtttcatcaatcttatgttttcctctactttatatttacaatagctcttttaatatccttgtctactaattccatcacctctgtcttttctgggtttctactgatttttctcctggttataagtcatattttattgcttctttgcataacacattagtttttttggatgccggacactgtaggtccagagtagcttttaatctagagttaattagctgcactactaaaacaaaacctttctgagaattctacctgatgctccatgtgtttccactctgtttccactctggctgctgagaacataaactattcccagccctgcatgagttccaggaattgttcagcctgctgctttccagtgcttcttttcctggcctcagtgcaagtcagtactaagtcaaaggactcaggggactcccagcagacttcttgagccctgtatctagaaggatcccatctctccagtactttcccctggaaattctagctgctgtggcctccccaactgccagtcctgtctcttcaattcagcgagatttattgtttcccttccctgaactgcaacctaggaactgccatgcgggggcaggctgagaaaccatggtgctcacctcactctgtctgcagtctcctgaggatcacaaacctgtgcttgtcctatgtctaaaaaccattacctattatacgtattgtatagcttccagttgtttaaggcaggagaggaaatctgacccttgttattccatcacagcagtaaggagaactcttcacatctaagtaaacacacctcacacttacaattcactgctttttgtaataattgatgtataaagaacaccacttccttacagaactatttcaatagcatcatgcttgtcaaattctttacattattgagactactcttcagtatgaacctctgtaggtattattctcaagtgtacagtgagttgtcctttcttgaaatcttccactttgttataaaaaacaatagaattttcttcctgtttaggtattctaaacatttaataaactgacttttgactaaaagcttctctactatcacaacactaataaggttttcacctcaatgagtcatccaatatgtaacgagtagtgtcttctgggagatgactttttttacactgtttgctttttaaaaacttctctttctaaattctgcttagtgactcttgactcctcaattcaagctttttcaacagtcactgcctcaatagggtttctctcccacatgcatcctcaaaagtgtcagaaagtatgacacttgatagcaacctttctgcattcgccaaagtcatgatttttatattatatgatttctctgatgtatcataagctgcgacttcctgttgaaggtggtcccacactcattgcatccatagtatttatctcctgtatgaatcctctgatgcctcataaggtgtgactttcttgtgaaagatttcccacattcaccacatttatatggtctctctcctgtatgaattctctgatgtataatcagctgtgccttctcaaagaaagcttttgcacaatcgctgcatccataggttttctctcctgtgtgatttctttgatgcttaatgagctgcactttctgaacaaatgctttcccacattcactgcattcatagggtttctcccctgtatgaattctctgatgcctaagaagctgtggcttccaggcaaaagctttcctacattcactacattcaaagggcttttctccagtatgggttctctgatgatgaatgagacttgacttctcactgaaggttttcctgcattcactgcattcatagggtttctcacctgtatgtgttctctgatgtgatatcaggcttgacttctgggtgaaggccttcccacactcactgcattcataaggcttctccccagtgtgtgttctgtgatgcgttaggagctgggacttcccaaagaaggttttcccacattgaatgcatccatatggtttctctcctaagtgaattttttgatgtcttattaactctgacttcttaaagaaggcctcctcacaatcactgcatcgatagttcttctctcctgtgtgagttatctgatgtttaatcagctgtggttttctgatgaaggcttcaccacattcgttgcattcgtagggcttctctcctgtatgaatcctctgatgcctaatgagaagtgagttcctgctgaaggctttttgacactcaccacatccgtaaggtttcttccctgtgtgggtcctctgatgagtaatcagctgcgacttccaaaagaaggcttttccacagtgactacatggatagggtttctctcctgtgtgcgctctctgatgtgtgatgagttttaatttctgggagaatgctttcccacactcactgcaactgtagggtttctctattgtgtgcgttatctgatgtcttttaagctgcgacttcctactgaaggcttttccacattcactgcatccatacggcttctctccagtatgaattctctgatgtaaaatgaggagtgacttcctactaaaagctttctgacattcgctgcacccatgcggtttttctcctgagtgagttctttgatgaaccgtgagcagtgacttctgtgaaaaggcttttccacactcactgcattgatagggcttctctcctgtatgagttctctggtgtataacaagttgtgacttcttgttaaaaaatctgccacattccatgcataaatagactcctgtgtgtgttatgtgattagcagtgagccatggctcttcgttgctggattttctacatgtactgcaatcacagtattttatcccaccatgggttctgccaggtttgatacagaacaataatttcttattgagttcatcaattttctttctttcacaattattttttggaataagcaaatcaaaaggacatttcaaacttttttctcctgtgccacatttatgggatcgcagtcctacatgaacaatgtttatgcttgaattaaatatttttccaaaaacatcatatttatggcctctctccatacttttaaggttgtcttgattatctcggagccacattttgggattatctagccagacttctgaaaagttctgatttaggatttcttgacctattatccatggatcttgttgttccagtttgaacattgcatcaggtttgagaatttgaaaacccaagaaaaccagattgctatagttctccaacatcacatctctgtacaagttcttctgagtaggattaagtagctgccattcctccagcgtgaaatccacagccacatcctcaaatgatatctgtgactggatcattttccgctgctcttgggaaatctgctgttttgtgacttctcttagtcctgacaccctggagtggcctctggtcagtggtctgtaaactgagaatacatccttggtcttgtgggctcttctttcttatctcacatgaattgtcttgttccagagggctattgcccctcggacctcgcagggccgcggcggacacggcccgatcggggacgtgaacgcgcagaactac

SEQ ID NO: 13765 - RNA, 696 nt, Homo sapiens
  source 1..696: mol_type = other RNA
gctgggattacaggcatgagccaccatgcccggcctaaacaattatttaataacattttcaggagcaaagaatatacacttaataaaaacaaccataaaatgccggtcttctttgatgactcccagggaattcactgtatttgaaatcatacattcatcaaatatttagttggcctgttcccggattatccatacacaaggaaatcaatgatccttcatcttcattcaaatgtgccataaaatcctctgggtccacaagtccccacgccatacttctttagagatgctaaagctgctgccttaaccctagggttatccaacaatccaagaaaattaaatgaggcgaagtttatacattcttttccattcaccacagttttgtggcttggagggcctgaaacgatgttgtagttgagagcaggatggtcttttgggacaggaggaacaagaggttctggttgccactcttcaatcagttcttctttttccttgactgtaagatcagatcgttcttgtaatttgtaagtcttagagaaaagaagtctgattatccagaggatcagaatcccttccaaaataagatggtaagcaggagcctcgtaaagcgcctgtaccatctccaccagaacccactgctccgtggcggtcgccatagttagccgcttccttccggaaggcgggtcacaagcgcgtccc

SEQ ID NO: 13766 - RNA, 2394 nt, Homo sapiens
  source 1..2394: mol_type = other RNA
gctgggattacaggcatgagccaccatgcccggcctacctttcagtgcccacttaactccattggttcagaggcactcagtgtatcagctgaaagggaattgatatgtgtcctgtgcaaagtactagtgctattgaggataggcttatccaaaaattggacttggggctggagaggtacatcttctagttccagcaatgtaattttgttgagggctcccctaggaaacagcaggaatcttggcacgtagagggtctgttgtggcccctgctttgtccagtaccggcccaagttaaacccattgatccagacttggcccttggtccatccaggtagatatagaaatgtgtccccaactgagcctaaaattggaaatgttttggagtagaatgtggggccagaaggagcttgaggatatggccattttggcaactggaggggaaaccaccacttcacaaggttatcaattttcagagggaacatcatccactgggtaaggattgtttgccccagaattggtggcttcaacaggcccttgaagtcactgctgttagacccaaagctgagcctccccatgttctccaccaagatatccagtttggaccccagtttccccgtcaaaaatagtttgtctctcatatttcgctccacaacaccctggaacaccccatccaccatcacataggcacggtcatggactccattatttggcacccagaatggtgttggctcaaaaatggtatgggtcatataggttcggtacaacatgaagccatggtcctgcttgacagcctcaaaggtcattggcaagattgaatgaatgggcccacgggggcaaagcaagtctaggaaagccagtaaatgcccaaccaggtgcagagtcacaggtccaagcatcatcttggggctcgggggaggtaaaggtcccaaaggaacttcctggaacttgctgatgacatctcgaagagcaaaaagcttaggtgtggggtcccctgcttcagatataggtgcatcatagtcatagctggtagtaatcggaaggaagcgtcccttcttatcggcaccattccaatatccaaagttggtacctccatggaacatgtacatgttcacactggctcccaacttgagcatgttctctagtcctttggttacagctgacacagaccgtgtggagtgattctggccccagtaatccagccagcctgtgtagtactcagagtttaccaatggcccatggggttcatacttccgaagcagggtaaagattttggtcatgttgtcagctgaatgctaatgatgttgcccccattgtgataaagccatggatatatcttgggcagcaagaccttgaaccaggagtccactgcggcaaggaagtctggatctgaggttcttagatgaatttcaggttttcgaagcaaccaggatgggagaccccccatctcccactctgcacagatgtaaggtcctggtctcagtatgaccaacaggttcgctagagctgcctcattcagaaaggcaatgaggtcccggctgccattaaagttatagaccccaggctgtggctcgtggtagttccagggcacataaaactgtatggcgttgaggccgctccatcgcatcttcaaaagccggtcggcccaaagcacccgcggtacccgaaagtagtgcaggctgccagacacatagcggaacggggccccgtctaggagaaaccggtcatgacccctatccactacgaacgaccgagtgtctgcctggggcagcagtagcgtcaggctgagcggcagcagcagggaacgaaggcaggacagcttcttgggagccatggcgtttacagcgctcctctagtctgagacggcggacagaccgtcacgtgtcggattcctgggagggaacctcagcgagcaagggggcggaaaccacctcaagttgccaggcgtttagcctggacttcctctccagcctgcagccacccccttactctactagtttgtaaaatttctacatcatgttaaagtgcagttcacgaaccagcttcatcgacatcacctgggaacttgttagaaatggagaatctggctgggcacgatggctcacgcctgtaatcccaacactttgggaggccgaggcgggtggatcacttgaggtcaggagttcaagaccagcttggccaacagggcaaaaccctgtctctactccaacattgggagatggaggtcctgggggcctcgggccgagcccggctttgctcccctttggcgtaggtgcctgcgtcttgacccccaccgaaggccaagtagagaaccctcaccagggtcctgggacccgtccacccctacacctagctagcccggagcctctcagctccgcgtccccacatcctccggat

SEQ ID NO: 13767 - RNA, 1794 nt, Homo sapiens
  source 1..1794: mol_type = other RNA
gctgggattacaggcatgagccaccatgcccggcctacctttcagtgcccacttaactccattggttcagaggcactcagtgtatcagctgaaagggaattgatatgtgtcctgtgcaaagtactagtgctattgaggataggcttatccaaaaattggacttggggctggagaggtacatcttctagttccagcaatgtaattttgttgagggctcccctaggaaacagcaggaatcttggcacgtagagggtctgttgtggcccctgctttgtccagtaccggcccaagttaaacccattgatccagacttggcccttggtccatccaggtagatatagaaatgtgtccccaactgagcctaaaattggaaatgttttggagtagaatgtggggccagaaggagcttgaggatatggccattttggcaactggaggggaaaccaccacttcacaaggttatcaattttcagagggaacatcatccactgggtaaggattgtttgccccagaattggtggcttcaacaggcccttgaagtcactgctgttagacccaaagctgagcctccccatgttctccaccaagatatccagtttggaccccagtttccccgtcaaaaatagtttgtctctcatatttcgctccacaacaccctggaacaccccatccaccatcacataggcacggtcatggactccattatttggcacccagaatggtgttggctcaaaaatggtatgggtcatataggttcggtacaacatgaagccatggtcctgcttgacagcctcaaaggtcattggcaagattgaatgaatgggcccacgggggcaaagcaagtctaggaaagccagtaaatgcccaaccaggtgcagagtcacaggtccaagcatcatcttggggctcgggggaggtaaaggtcccaaaggaacttcctggaacttgctgatgacatctcgaagagcaaaaagcttaggtgtggggtcccctgcttcagatataggtgcatcatagtcatagctggtagtaatcggaaggaagcgtcccttcttatcggcaccattccaatatccaaagttggtacctccatggaacatgtacatgttcacactggctcccaacttgagcatgttctctagtcctttggttacagctgacacagaccgtgtggagtgattctggccccagtaatccagccagcctgtgtagtactcagagtttaccaatggcccatggggttcatacttccgaagcagggtaaagattttggtcatgttgtcagctggatctgaggttcttagatgaatttcaggttttcgaagcaaccaggatgggagaccccccatctcccactctgcacagatgtaaggtcctggtctcagtatgaccaacaggttcgctagagctgcctcattcagaaaggcaatgaggtcccggctgccattaaagttatagaccccaggctgtggctcgtggtagttccagggcacataaaactgtatggcgttgaggccgctccatcgcatcttcaaaagccggtcggcccaaagcacccgcggtacccgaaagtagtgcaggctgccagacacatagcggaacggggccccgtctaggagaaaccggtcatgacccctatccactacgaacgaccgagtgtctgcctggggcagcagtagcgtcaggctgagcggcagcagcagggaacgaaggcaggacagcttcttgggagccatggcgtttacagcgctcctctagtctgagacggcggacagaccgtcacgtgtcggattc

SEQ ID NO: 13768 - RNA, 1961 nt, Homo sapiens
  source 1..1961: mol_type = other RNA
gctgggattacaggcatgagccaccatgcccggcctacctttcagtgcccacttaactccattggttcagaggcactcagtgtatcagctgaaagggaattgatatgtgtcctgtgcaaagtactagtgctattgaggataggcttatccaaaaattggacttggggctggagaggtacatcttctagttccagcaatgtaattttgttgagggctcccctaggaaacagcaggaatcttggcacgtagagggtctgttgtggcccctgctttgtccagtaccggcccaagttaaacccattgatccagacttggcccttggtccatccaggtagatatagaaatgtgtccccaactgagcctaaaattggaaatgttttggagtagaatgtggggccagaaggagcttgaggatatggccattttggcaactggaggggaaaccaccacttcacaaggttatcaattttcagagggaacatcatccactgggtaaggattgtttgccccagaattggtggcttcaacaggcccttgaagtcactgctgttagacccaaagctgagcctccccatgttctccaccaagatatccagtttggaccccagtttccccgtcaaaaatagtttgtctctcatatttcgctccacaacaccctggaacaccccatccaccatcacataggcacggtcatggactccattatttggcacccagaatggtgttggctcaaaaatggtatgggtcatataggttcggtacaacatgaagccatggtcctgcttgacagcctcaaaggtcattggcaagattgaatgaatgggcccacgggggcaaagcaagtctaggaaagccagtaaatgcccaaccaggtgcagagtcacaggtccaagcatcatcttggggctcgggggaggtaaaggtcccaaaggaacttcctggaacttgctgatgacatctcgaagagcaaaaagcttaggtgtggggtcccctgcttcagatataggtgcatcatagtcatagctggtagtaatcggaaggaagcgtcccttcttatcggcaccattccaatatccaaagttggtacctccatggaacatgtacatgttcacactggctcccaacttgagcatgttctctagtcctttggttacagctgacacagaccgtgtggagtgattctggccccagtaatccagccagcctgtgtagtactcagagtttaccaatggcccatggggttcatacttccgaagcagggtaaagattttggtcatgttgtcagctggatctgaggttcttagatgaatttcaggttttcgaagcaaccaggatgggagaccccccatctcccactctgcacagatgtaaggtcctggtctcagtatgaccaacaggttcgctagagctgcctcattcagaaaggcaatgaggtcccggctgccattaaagttatagaccccaggctgtggctcgtggtagttccagggcacataaaactgtatggcgttgaggccgctccatcgcatcttcaaaagccggtcggcccaaagcacccgcggtacccgaaagtagtgcaggctgccagacacatagcggaacggggccccgtctaggagaaaccggtcatgacccctatccactacgaacgaccgagtgtctgcctggggcagcagtagcgtcaggctgagcggcagcagcagggaacgaaggcaggacagcttcttgggagccatggcgtttacagcgctcctctagtctgagacggcggacagaccgtcacgtgtcggattcctccaacattgggagatggaggtcctgggggcctcgggccgagcccggctttgctcccctttggcgtaggtgcctgcgtcttgacccccaccgaaggccaagtagagaaccctcaccagggtcctgggacccgtccacccctacacctagctagcccggagcctctc

SEQ ID NO: 13769 - RNA, 2318 nt, Homo sapiens
  source 1..2318: mol_type = other RNA
gctgggattacaggcatgagccaccatgcccggcctacctttcagtgcccacttaactccattggttcagaggcactcagtgtatcagctgaaagggaattgatatgtgtcctgtgcaaagtactagtgctattgaggataggcttatccaaaaattggacttggggctggagaggtacatcttctagttccagcaatgtaattttgttgagggctcccctaggaaacagcaggaatcttggcacgtagagggtctgttgtggcccctgctttgtccagtaccggcccaagttaaacccattgatccagacttggcccttggtccatccaggtagatatagaaatgtgtccccaactgagcctaaaattggaaatgttttggagtagaatgtggggccagaaggagcttgaggatatggccattttggcaactggaggggaaaccaccacttcacaaggttatcaattttcagagggaacatcatccactgggtaaggattgtttgccccagaattggtggcttcaacaggcccttgaagtcactgctgttagacccaaagctgagcctccccatgttctccaccaagatatccagtttggaccccagtttccccgtcaaaaatagtttgtctctcatatttcgctccacaacaccctggaacaccccatccaccatcacataggcacggtcatggactccattatttggcacccagaatggtgttggctcaaaaatggtatgggtcatataggttcggtacaacatgaagccatggtcctgcttgacagcctcaaaggtcattggcaagattgaatgaatgggcccacgggggcaaagcaagtctaggaaagccagtaaatgcccaaccaggtgcagagtcacaggtccaagcatcatcttggggctcgggggaggtaaaggtcccaaaggaacttcctggaacttgctgatgacatctcgaagagcaaaaagcttaggtgtggggtcccctgcttcagatataggtgcatcatagtcatagctggtagtaatcggaaggaagcgtcccttcttatcggcaccattccaatatccaaagttggtacctccatggaacatgtacatgttcacactggctcccaacttgagcatgttctctagtcctttggttacagctgacacagaccgtgtggagtgattctggccccagtaatccagccagcctgtgtagtactcagagtttaccaatggcccatggggttcatacttccgaagcagggtaaagattttggtcatgttgtcagctggatctgaggttcttagatgaatttcaggttttcgaagcaaccaggatgggagaccccccatctcccactctgcacagatgtaaggtcctggtctcagtatgaccaacaggttcgctagagctgcctcattcagaaaggcaatgaggtcccggctgccattaaagttatagaccccaggctgtggctcgtggtagttccagggcacataaaactgtatggcgttgaggccgctccatcgcatcttcaaaagccggtcggcccaaagcacccgcggtacccgaaagtagtgcaggctgccagacacatagcggaacggggccccgtctaggagaaaccggtcatgacccctatccactacgaacgaccgagtgtctgcctggggcagcagtagcgtcaggctgagcggcagcagcagggaacgaaggcaggacagcttcttgggagccatggcgtttacagcgctcctctagtctgagacggcggacagaccgtcacgtgtcggattcctgggagggaacctcagcgagcaagggggcggaaaccacctcaagttgccaggcgtttagcctggacttcctctccagcctgcagccacccccttactctactagtttgtaaaatttctacatcatgttaaagtgcagttcacgaaccagcttcatcgacatcacctgggaacttgttagaaatggagaatctggctgggcacgatggctcacgcctgtaatcccaacactttgggaggccgaggcgggtggatcacttgaggtcaggagttcaagaccagcttggccaacagggcaaaaccctgtctctactccaacattgggagatggaggtcctgggggcctcgggccgagcccggctttgctcccctttggcgtaggtgcctgcgtcttgacccccaccgaaggccaagtagagaaccctcaccagggtcctgggacccgtccacccctacacctagctagcccggagcctctcagctccgcgtccccacatcctccggatgcccagcggttgctgagat

SEQ ID NO: 13770 - RNA, 2280 nt, Homo sapiens
  source 1..2280: mol_type = other RNA
gctgggattacaggcatgagccaccatgcccggcctacctttcagtgcccacttaactccattggttcagaggcactcagtgtatcagctgaaagggaattgatatgtgtcctgtgcaaagtactagtgctattgaggataggcttatccaaaaattggacttggggctggagaggtacatcttctagttccagcaatgtaattttgttgagggctcccctaggaaacagcaggaatcttggcacgtagagggtctgttgtggcccctgctttgtccagtaccggcccaagttaaacccattgatccagacttggcccttggtccatccaggtagatatagaaatgtgtccccaactgagcctaaaattggaaatgttttggagtagaatgtggggccagaaggagcttgaggatatggccattttggcaactggaggggaaaccaccacttcacaaggttatcaattttcagagggaacatcatccactgggtaaggattgtttgccccagaattggtggcttcaacaggcccttgaagtcactgctgttagacccaaagctgagcctccccatgttctccaccaagatatccagtttggaccccagtttccccgtcaaaaatagtttgtctctcatatttcgctccacaacaccctggaacaccccatccaccatcacataggcacggtcatggactccattatttggcacccagaatggtgttggctcaaaaatggtatgggtcatataggttcggtacaacatgaagccatggtcctgcttgacagcctcaaaggtcattggcaagattgaatgaatgggcccacgggggcaaagcaagtctaggaaagccagtaaatgcccaaccaggtgcagagtcacaggtccaagcatcatcttggggctcgggggaggtaaaggtcccaaaggaacttcctggaacttgctgatgacatctcgaagagcaaaaagcttaggtgtggggtcccctgcttcagatataggtgcatcatagtcatagctggtagtaatcggaaggaagcgtcccttcttatcggcaccattccaatatccaaagttggtacctccatggaacatgtacatgttcacactggctcccaacttgagcatgttctctagtcctttggttacagctgacacagaccgtgtggagtgattctggccccagtaatccagccagcctgtgtagtactcagagtttaccaatggcccatggggttcatacttccgaagcagggtaaagattttggtcatgttgtcagctgggccaaaatctacagtggtatagagtccccggagggagccacacttgagtccttcaggcccatctgtggtgaagagcaagatcttttctcctagcagtgcacggaagagcccagccaagtgcctcatgtagctgaagtcacaggctctgtagctaccatattcattctccacctgaatgctaatgatgttgcccccattgtgataaagccatggatatatcttgggcagcaagaccttgaaccaggagtccactgcggcaaggaagtctggatctgaggttcttagatgaatttcaggttttcgaagcaaccaggatgggagaccccccatctcccactctgcacagatgtaaggtcctggtctcagtatgaccaacaggttcgctagagctgcctcattcagaaaggcaatgaggtcccggctgccattaaagttatagaccccaggctgtggctcgtggtagttccagggcacataaaactgtatggcgttgaggccgctccatcgcatcttcaaaagccggtcggcccaaagcacccgcggtacccgaaagtagtgcaggctgccagacacatagcggaacggggccccgtctaggagaaaccggtcatgacccctatccactacgaacgaccgagtgtctgcctggggcagcagtagcgtcaggctgagcggcagcagcagggaacgaaggcaggacagcttcttgggagccatggcgtttacagcgctcctctagtctgagacggcggacagaccgtcacgtgtcggattcctccaacattgggagatggaggtcctgggggcctcgggccgagcccggctttgctcccctttggcgtaggtgcctgcgtcttgacccccaccgaaggccaagtagagaaccctcaccagggtcctgggacccgtccacccctacacctagctagcccggagcctctcagctccgcgtccccacatcctccggatgcccagcggttgctgagatacc

SEQ ID NO: 13771 - RNA, 2569 nt, Homo sapiens
  source 1..2569: mol_type = other RNA
gctgggattacaggcatgagccaccatgcccggcctacctttcagtgcccacttaactccattggttcagaggcactcagtgtatcagctgaaagggaattgatatgtgtcctgtgcaaagtactagtgctattgaggataggcttatccaaaaattggacttggggctggagaggtacatcttctagttccagcaatgtaattttgttgagggctcccctaggaaacagcaggaatcttggcacgtagagggtctgttgtggcccctgctttgtccagtaccggcccaagttaaacccattgatccagacttggcccttggtccatccaggtagatatagaaatgtgtccccaactgagcctaaaattggaaatgttttggagtagaatgtggggccagaaggagcttgaggatatggccattttggcaactggaggggaaaccaccacttcacaaggttatcaattttcagagggaacatcatccactgggtaaggattgtttgccccagaattggtggcttcaacaggcccttgaagtcactgctgttagacccaaagctgagcctccccatgttctccaccaagatatccagtttggaccccagtttccccgtcaaaaatagtttgtctctcatatttcgctccacaacaccctggaacaccccatccaccatcacataggcacggtcatggactccattatttggcacccagaatggtgttggctcaaaaatggtatgggtcatataggttcggtacaacatgaagccatggtcctgcttgacagcctcaaaggtcattggcaagattgaatgaatgggcccacgggggcaaagcaagtctaggaaagccagtaaatgcccaaccaggtgcagagtcacaggtccaagcatcatcttggggctcgggggaggtaaaggtcccaaaggaacttcctggaacttgctgatgacatctcgaagagcaaaaagcttaggtgtggggtcccctgcttcagatataggtgcatcatagtcatagctggtagtaatcggaaggaagcgtcccttcttatcggcaccattccaatatccaaagttggtacctccatggaacatgtacatgttcacactggctcccaacttgagcatgttctctagtcctttggttacagctgacacagaccgtgtggagtgattctggccccagtaatccagccagcctgtgtagtactcagagtttaccaatggcccatggggttcatacttccgaagcagggtaaagattttggtcatgttgtcagctgggccaaaatctacagtggtatagagtccccggagggagccacacttgagtccttcaggcccatctgtggtgaagagcaagatcttttctcctagcagtgcacggaagagcccagccaagtgcctcatgtagctgaagtcacaggctctgtagctaccatattcattctccacctgaatgctaatgatgttgcccccattgtgataaagccatggatatatcttgggcagcaagaccttgaaccaggagtccactgcggcaaggaagtctggatctgaggttcttagatgaatttcaggttttcgaagcaaccaggatgggagaccccccatctcccactctgcacagatgtaaggtcctggtctcagtatgaccaacaggttcgctagagctgcctcattcagaaaggcaatgaggtcccggctgccattaaagttatagaccccaggctgtggctcgtggtagttccagggcacataaaactgtatggcgttgaggccgctccatcgcatcttcaaaagccggtcggcccaaagcacccgcggtacccgaaagtagtgcaggctgccagacacatagcggaacggggccccgtctaggagaaaccggtcatgacccctatccactacgaacgaccgagtgtctgcctggggcagcagtagcgtcaggctgagcggcagcagcagggaacgaaggcaggacagcttcttgggagccatggcgtttacagcgctcctctagtctgagacggcggacagaccgtcacgtgtcggattcctgggagggaacctcagcgagcaagggggcggaaaccacctcaagttgccaggcgtttagcctggacttcctctccagcctgcagccacccccttactctactagtttgtaaaatttctacatcatgttaaagtgcagttcacgaaccagcttcatcgacatcacctgggaacttgttagaaatggagaatctggctgggcacgatggctcacgcctgtaatcccaacactttgggaggccgaggcgggtggatcacttgaggtcaggagttcaagaccagcttggccaacagggcaaaaccctgtctctactccaacattgggagatggaggtcctgggggcctcgggccgagcccggctttgctcccctttggcgtaggtgcctgcgtcttgacccccaccgaaggccaagtagagaaccctcaccagggtcctgggacccgtccacccctacacctagctagcccggagcctctcagctccgcgtccccacatcctccggat

SEQ ID NO: 13772 - RNA, 2292 nt, Homo sapiens
  source 1..2292: mol_type = other RNA
gctgggattacaggcatgagccaccatgcccggcctacctttcagtgcccacttaactccattggttcagaggcactcagtgtatcagctgaaagggaattgatatgtgtcctgtgcaaagtactagtgctattgaggataggcttatccaaaaattggacttggggctggagaggtacatcttctagttccagcaatgtaattttgttgagggctcccctaggaaacagcaggaatcttggcacgtagagggtctgttgtggcccctgctttgtccagtaccggcccaagttaaacccattgatccagacttggcccttggtccatccaggtagatatagaaatgtgtccccaactgagcctaaaattggaaatgttttggagtagaatgtggggccagaaggagcttgaggatatggccattttggcaactggaggggaaaccaccacttcacaaggttatcaattttcagagggaacatcatccactgggtaaggattgtttgccccagaattggtggcttcaacaggcccttgaagtcactgctgttagacccaaagctgagcctccccatgttctccaccaagatatccagtttggaccccagtttccccgtcaaaaatagtttgtctctcatatttcgctccacaacaccctggaacaccccatccaccatcacataggcacggtcatggactccattatttggcacccagaatggtgttggctcaaaaatggtatgggtcatataggttcggtacaacatgaagccatggtcctgcttgacagcctcaaaggtcattggcaagattgaatgaatgggcccacgggggcaaagcaagtctaggaaagccagtaaatgcccaaccaggtgcagagtcacaggtccaagcatcatcttggggctcgggggaggtaaaggtcccaaaggaacttcctggaacttgctgatgacatctcgaagagcaaaaagcttaggtgtggggtcccctgcttcagatataggtgcatcatagtcatagctggtagtaatcggaaggaagcgtcccttcttatcggcaccattccaatatccaaagttggtacctccatggaacatgtacatgttcacactggctcccaacttgagcatgttctctagtcctttggttacagctgacacagaccgtgtggagtgattctggccccagtaatccagccagcctgtgtagtactcagagtttaccaatggcccatggggttcatacttccgaagcagggtaaagattttggtcatgttgtcagctgggccaaaatctacagtggtatagagtccccggagggagccacacttgagtccttcaggcccatctgtggtgaagagcaagatcttttctcctagcagtgcacggaagagcccagccaagtgcctcatgtagctgaagtcacaggctctgtagctaccatattcattctccacctgaatgctaatgatgttgcccccattgtgataaagccatggatatatcttgggcagcaagaccttgaaccaggagtccactgcggcaaggaagtctggatctgaggttcttagatgaatttcaggttttcgaagcaaccaggatgggagaccccccatctcccactctgcacagatgtaaggtcctggtctcagtatgaccaacaggttcgctagagctgcctcattcagaaaggcaatgaggtcccggctgccattaaagttatagaccccaggctgtggctcgtggtagttccagggcacataaaactgtatggcgttgaggccgctccatcgcatcttcaaaagccggtcggcccaaagcacccgcggtacccgaaagtagtgcaggctgccagacacatagcggaacggggccccgtctaggagaaaccggtcatgacccctatccactacgaacgaccgagtgtctgcctggggcagcagtagcgtcaggctgagcggcagcagcagggaacgaaggcaggacagcttcttgggagccatggcgtttacagcgctcctctagtctgagacggcggacagaccgtcacgtgtcggattcctgggagggaacctccaacattgggagatggaggtcctgggggcctcgggccgagcccggctttgctcccctttggcgtaggtgcctgcgtcttgacccccaccgaaggccaagtagagaaccctcaccagggtcctgggacccgtccacccctacacctagctagcccggagcctctcagctccgcgtccccacatcctccggatgcccagcggttgctgagatacc

SEQ ID NO: 13773 - RNA, 869 nt, Homo sapiens
  source 1..869: mol_type = other RNA
gctgggattacaggcatgagccaccatgcccggcctatcaaataacacaaatttcttataccaaaatgacaaggtagtcagtgagatgggagagacatagattttttaaataccctaaatccttttgtgtgcccaggatatggtggtggtggtgaaacactgtgttttctggtcagcgccactgcctgttcataagaaggtaatcctgcatcctccacagaaggcggcaatggagacaaggcagcctcctcaggtcttctgaaaatgatggagggagtgtgcctccccctttcatagacggctgaagagcatggatgttgtagcctattacacttagtgatacaaagatagtagccaagtaatccaaaaataaccaaaaatactccagcagcaattaatccagtcagaaggcccataacatctattttctctctgttgccatctgattttgtggttggtcctttagctgaatattcctgccaaaatgcaatcgttttatcttcatccacaaaaatctctctggcttcctcataattgcaaagttcttcattgcactctctttctaggttgccgggagtgaagagctccagatcaaatctattatacagaaggcgtctatgtatgaaaaagtttgcttcttcttttgatgtaaacacttcttctcccgcatgcttagaagcctttggacctcttgcgcaatgaggaaaccccagggtaactgtgggcagttggctgagtagaaccagaagcgtaaacatagtctggcaactgtcaaacaaactgcggcgagcgggcgggcagtgggccggcgtctcccgggagcccgcgctgcgctctcagccgccccagcttctgccccatccccgggc

SEQ ID NO: 13774 - RNA, 1027 nt, Homo sapiens
  source 1..1027: mol_type = other RNA
gctgggattacaggcatgagccaccatgcccggcctatcaaataacacaaatttcttataccaaaatgacaaggtagtcagtgagatgggagagacatagattttttaaataccctaaatccttttgtgtgcccaggatatggtggtggtggtgaaacactgtgttttctggtcagcgccactgcctgttcataagaaggtaatcctgcatcctccacagaaggcggcaatggagacaaggcagcctcctcaggtcttctgaaaatgatggagggagtgtgcctccccctttcatagacggctgaagagcatggatgttgtagcctattacacttagtgatacaaagatagtagccaagtaatccaaaaataaccaaaaatactccagcagcaattaatccagtcagaaggcccataacatctattttctctctgttgccatctgattttgtggttggtcctttagctgaatattcctgccaaaatgcaatcgttttatcttcatccacaaaaatctctctggcttcctcataattgcaaagttcttcattgcactctctttctaggttgccgggagtgaagagctccagatcaaatctattatacagaaggcgtctatgtatgaaaaagtttgcttcttcttttgatgtaaacacttcttctcccgcatgcttagaagcctttggacctcttgcgcaatgaggaaaccccagggtaactgtgggcagttggctgagtagaaccagaagcgtaaacatagtctggcaactgtcaaacaaactgtgtccccccgcacatgttccagcagcccccgggccagaggctcttcttggggcggttccttcggccgccaggccctcggtctccggcgccctcaaacctcggcgacgctccgggcctcgctctccgcagggtctggatggcccccgcgcgcaaacctgggaagggcctggggttcgcagaggggcgcccggggaacacgcgcggggtgaggtcctgcctcggtccggggaggcggccgacggag

SEQ ID NO: 13775 - RNA, 2114 nt, Homo sapiens
  source 1..2114: mol_type = other RNA
gctgggattacaggcatgagccaccatgcccggcctcccagttttcatgatgaggaagtgatggtagcttttcatctgcccagaagttaacttttgatggatttgccttctaaggcatcaaacatgtcttctaaggccttctccacacattggagaaactcccgggcattgcggcctgggtaggaagagacattgcagcctatccagttgtcatgaacagcatacccaacaccaaagccatcagagaccacaggggcaaagcccccaaggttcactgctgggctgctcagtgtgctcgtggacaggacattgtggtttatctgcccgtatgcagggtccaggtagagctcaggcaagatgatccctttggctgctgccagatgccgcagagcaaacaagtgtcggtcaaagccctggccagcactgtgcctggagggctccctgacaaaggcctcagagcacctctttgtatagacggaggccgggcggatggtctcagtgcggccgtgcttgaatgcggcagtgctacaggactcgtaggtggccactgtctgcccgtactgccgcaggaaggccatctggaatgccagctgggcaactgcgtcagggctcagcttttgcttcttcaggaattctttgcctcctctctgaaactggacgcagtcaatagtgagggttttcatggtggcatcaaacttttccttagcagctgtgatgccagtctttaaggcatcagtcagctcgaagttgagtttctgcaccgtgacagtagagtcagtggtagctggctggctctgtggagtgacggcaggggtctgagtgctgtctttaaatacttcattaaaaaatctgagcactgccacaccatcaccccaagagtgctcaaagtggacggcagtagagccatccttggcgataatgaggttaaaggatttatcaaaccagcggtttgtgccatccccatgcagcatattgtgggacaagtggacaaggtccttaatggggaagtcatctaggcagagacagaacactgccgagtccactttcctcaggctctcctcattgccactactcatcagcttctgcctgagctctgcccagatgtctcggttctcactggtcaggtatgccaggggaaactcgggggcggggctgctgtctgagagaatgtacttcagatgtgcctggatttccgaggggctcacaatgttcccatcttgatccaggacatcaaagatataaaaatttcctttccttaggaccaggaggtgtctggccttgtcatcagtgaagagttcatcccgactgggtttgggtaaacgagttgagttgaaaagccgaaaatactgggacatatccaggggatacgcattgaccaggtaggccccataccaggacagagaggaaggcacaaagcgtatgagtctcttgaaggtgatagtgtcactttttgcagggttcaagtggaacacttctggctccagaaggccagcccggagtgtcttcagaaaccggatggcagaaacagtcatgttggttgcccgggtgagctggtcattatactcagattttgggtcaggattgaaagccataaatggattaaagttcagaacaacggagtctcgagcagataggtacatatcaaaccagggtcccgaaatgtagcttgtatgtttattctgtttgtccagagcaaccagctgctcatgcagttcttttccaatcccattttcaaaactcttgcaaaattgttctgttttcctgaactggccatcattcaagagaggcttctgtgcactgaggtatctcctaatggtgtcttcaagtttgggaataggcagcctgggcaggctgtcctggtagtgcatggtgggcacgatgctgcgctgcaggtactggccgggcccggagccggcgctgaggggccgactgggggctcccggaccaaccgcggggccccggggccaggcgcgcagcagcaggcggggcaccatcgtcccgggagcctgcggcggcgagaacgcggcaagtggggagttctggagtctaaacacaaggccgccgccgccgttagcgcccaagacactgcgtcaggactcctgaggcacttctcc

SEQ ID NO: 13776 - RNA, 2183 nt, Homo sapiens
  source 1..2183: mol_type = other RNA
gctgggattacaggcatgagccaccatgcccggcctcccagttttcatgatgaggaagtgatggtagcttttcatctgcccagaagttaacttttgatggatttgccttctaaggcatcaaacatgtcttctaaggccttctccacacattggagaaactcccgggcattgcggcctgggtaggaagagacattgcagcctatccagttgtcatgaacagcatacccaacaccaaagccatcagagaccacaggggcaaagcccccaaggttcactgctgggctgctcagtgtgctcgtggacaggacattgtggtttatctgcccgtatgcagggtccaggtagagctcaggcaagatgatccctttggctgctgccagatgccgcagagcaaacaagtgtcggtcaaagccctggcccattgctgcttctttggtcagctggccatggtacttggagcactcaaccatcatctgctgaagctcaccagcactgtgcctggagggctccctgacaaaggcctcagagcacctctttgtatagacggaggccgggcggatggtctcagtgcggccgtgcttgaatgcggcagtgctacaggactcgtaggtggccactgtctgcccgtactgccgcaggaaggccatctggaatgccagctgggcaactgcgtcagggctcagcttttgcttcttcaggaattctttgcctcctctctgaaactggacgcagtcaatagtgagggttttcatggtggcatcaaacttttccttagcagctgtgatgccagtctttaaggcatcagtcagctcgaagttgagtttctgcaccgtgacagtagagtcagtggtagctggctggctctgtggagtgacggcaggggtctgagtgctgtctttaaatacttcattaaaaaatctgagcactgccacaccatcaccccaagagtgctcaaagtggacggcagtagagccatccttggcgataatgaggttaaaggatttatcaaaccagcggtttgtgccatccccatgcagcatattgtgggacaagtggacaaggtccttaatggggaagtcatctaggcagagacagaacactgccgagtccactttcctcaggctctcctcattgccactactcatcagcttctgcctgagctctgcccagatgtctcggttctcactggtcaggtatgccaggggaaactcgggggcggggctgctgtctgagagaatgtacttcagatgtgcctggatttccgaggggctcacaatgttcccatcttgatccaggacatcaaagatataaaaatttcctttccttaggaccaggaggtgtctggccttgtcatcagtgaagagttcatcccgactgggtttgggtaaacgagttgagttgaaaagccgaaaatactgggacatatccaggggatacgcattgaccaggtaggccccataccaggacagagaggaaggcacaaagcgtatgagtctcttgaaggtgatagtgtcactttttgcagggttcaagtggaacacttctggctccagaaggccagcccggagtgtcttcagaaaccggatggcagaaacagtcatgttggttgcccgggtgagctggtcattatactcagattttgggtcaggattgaaagccataaatggattaaagttcagaacaacggagtctcgagcagataggtacatatcaaaccagggtcccgaaatgtagcttgtatgtttattctgtttgtccagagcaaccagctgctcatgcagttcttttccaatcccattttcaaaactcttgcaaaattgttctgttttcctgaactggccatcattcaagagaggcttctgtgcactgaggtatctcctaatggtgtcttcaagtttgggaataggcagcctgggcaggctgtcctggtagtgcatggtgggcacgatgctgcgctgcaggtactggccgggcccggagccggcgctgaggggccgactgggggctcccggaccaaccgcggggccccggggccaggcgcgcagcagcaggcggggcaccatcgtcccgggagcctgcggcggcgagaacgcggcaagtggggagttctggagtctaaacacaaggccgccgccgccgttagcgcccaagacactgcgtcaggactcctgaggcacttctcc

SEQ ID NO: 13777 - RNA, 3848 nt, Homo sapiens
  source 1..3848: mol_type = other RNA
gctgggattacaggcatgagccaccatgcccggcctgctttctcagtttggatctttaagctccaaccccagaagcatgaaagtcacacatgttaaaaaatactgtttaattttctagtaatgtcctttaaaaaaagctgatacattgagatttttttttaatcttctcagatctgcctctgaaaccactgcaaagcagctatgcaacttaatttttcagtactcatatatgtattaatggaggaaaagccactctgaggaagcacgccaaggacatgtccccacgtgggcacaccccatcagcactgggtacccaggaatgtgaatgcaaccctggcatgttcacagctaacattatgcccttgcattcttttttgctgtgaggaacaatatgatcacacagcactgaaaacggtagacacaaagggcctgcctttttctttctcatttttgcctttccagcttgcacttctattcctactccagtgacccatttattccccagttacccataatgaaaaatagttctgtcatttactgagccttacattcaaatgcaaatgacggactttataaaactgctgccaataaggtacaatgttcattgatacaatacgtttcaactgcaggtatgttgagcacacaagcaatcaccgtattgtattagagacattttattgaaaatgcgaaaataggaaatgtattatagcctaaaataaattacataacatatacagcatatatttatatctttaaaatatttttttttttaggttctttcagtctaggaattctgactaaatcaatttagtgaaccgtgtctataatttttttaaaggaaaaaacctgctttccaaaacttagaaaaatatactgcactgcatggatttcgaatgcgttatttcagggaggaccacatagtgactctggtatcgttataaaatgtcttgctttatcgtatggtgtgggagggaagtaccgtagtacattctcaattacctgtaccgcagagttatgactaaggatagcagaaccaggtaatatatctacttcaaaagttaccctacagcaacctggcattagaatgctggatgagacttaaagcttcagttcactgtaaaaactaaaatgcaaagttaggatgctccatgtgactcgctctaatgcgaccttcaggaaaggcgagggaaaagcaagccttcaggaaaagtcatgcggcagggtctggaatctggagatgcgcttttgtgacaatttaaaaaagttagctcatgtatatacacggtgggggtgagaactgacagcttgctcagatctaggagaacgcagagtgaaatgctatcattcaaccatgtcagtttgctgcccccggggcatttcaaaccaaacctttctacgggagattctgtccatctgtcagcctgctgtggtcacaggtctccgttcctcagtgtgaacggggactccgggctgcagcgtgccacccgcctcctgcatgtgtggagtagatggtttcgaactccgtggcggaagggaaatttaagaggccaccggggctccatctctttgtacggccatgtgactgggaagcaaatcaaaggaagccgagttttaacctgttgattcttaagagcgatgaagggggacaggagagtctgtggcctgctgtgcagggtgaccgaggcgcgatggcacagctgcagtcctttggttccaagaggagattgtccaggggaggaggacacaacgtcaaccgtgaggcagctgtgtcttttgggttttcgtgaggcaggggtatgaagtcagttgtttcgtttgtttttacatagcaacagtaaagaccattcactaggtccccccgtcagtgtgagcatacccagtatgctagagaattgacacgaaacctttaaatcaaggcctctttcattaccaaaacaaaacaaaaaaaagggaacaaaatacgatgggagagggaagagatgatgccgaagtgtcatcctgactgactgtccctgcagtgcccatggcgtcccgtgccttattcattctcctctctcatttccacgatgtctgtcacctcctctgtcggaggcatgtctgtcatggcagagtcttccccctccgtggccgactcattctccatcttctttttctgcttccggtagacatagcacgcagcgatggcgaccatggtggattctcccacaaagcccgccaggagggagcccacgcccagggtcgcaccgtgcacccccaggtagggtaggaccacgaggctggcgatgaggacgatgatccgcagcacagagctgggggcaaggacgaaggttttcttcagtgtcatcagccacccggtgagatgcgccctcactgtgactggaactgggaagaaggagaagatccgcaaaggaacaacacagagttctgcaaaggcaaagtccactccgatgatgtctatcaagattttctcagacacgttgggtgtccaaaacatcacgaaacagagcgtgagtgacagagccatgcagacgaaggtgaacttcttgatgtgggctgccgtgactgtgttgctcgtgctcaccagtttgttgctggggttattcttgtcgaaagcaggatacacagcacggatttccgtcaaccagccgtatggcatgtgacccacagggtatgtggctgtcaaaatcgccactgcctctgtggctgcagaactgccaccaaggtcccgggaaacaaagaggttgacaataggccgactgattctctgtgtggccagaattagagccaaaggccaccagaagctcagcatctttcttattgttgcatctccccccagctccgggccacttctgtcagggatgatgtcgtgaatgttcttgtagtagcccaggcacagggtggtgcagcgcacaagtgcgcccatgtacaaggagaggatcgggatgagcaggggctcccggcattccaggtgactgtgaagcaaaatggctacaaaaacaacctgagctatgacatctgagattgaggcacatcccaccaggaaactgtatttgtgttttaagagaatgccagcatgggtccatgccattgcgtccatgaaaggaaaggcggcgaggtacaggaaggcccttctcgtcttgctccccaccgactcgtccacatggtgcagtttattgataatgtagtatcctaaatcactataagctatcagtgtgtgaaagacggcagcgatggcccctgccaccaccatacacaggacggctttggtcctgtctctcttgctgttcacaaacaccaggcccacatttttgaagtcactcatgggacccgtgaagaacttcatgagggagtacgccagcccgtagctggccagcatctcgactgcatcctccttgacagcagcaatgccccggttcaaggcctgctccccgaagtcgatggctatgttggtgatgcccaggggcaccaagaaccggatcaggggccagtagtgcgtgagcgccgggaatttcaccatagtccccgccgtgggctgaccccacacacatctgctgccgcgaggggactctgcggggaggcgaggggcgacggggcgacggggcgagcggggcgcgggccgacagaggccgcgggcggcggggcctcgggcgcggcggcggcggctcctcctcgcggctgcggcgccttctccgagcgcggctgctctagcaggggatccgcaagctcaagtccatccctgctgccctcccacacaacaaagatctgccgggaaaaaaaagaggagggacggcggcggcggcggcggcggcagaaggttctgctgacagcggctccattataagcgctct

SEQ ID NO: 13778 - RNA, 1862 nt, Homo sapiens
  source 1..1862: mol_type = other RNA
gctgggattacaggcatgagccaccatgcccggcctggttgtggaacttcacgggaatttattttgtcattacaatgttggcaagatatttttttcgtgtgctgtaaactgaggttctgtcttggagtttatgtcatgtcaccaggtcctgtgctgaagggcatttgcacatcttttgtggcttctctcaggaaaatgtgggccttggcgacatccaatgctagtgctattccccttctcccctagagttacagaattataaccaccaggggacacctacaggccaggccaggccaggatcctggtgctgcttcagcctactgtggcctggaagggtccctgcctgctgaggcctaagatcctgacttggctaaaggaggggagggggcaggctgtggtatctagggtccatccccgcatcctgctcggtgccacctgacagatgtcatgccccaggtaggtatgtgccctgaaccttgccgggtgcacgtgcctgaacgtggcaccgtacccagctgggtaaaaacggctcgagcacggaagccaaaggatggattgccaaaacaaagattacgataatgtcaagtttaatctgccaaatatacaagttgaatttgtggagcatgttttgcctgggtgccacacagtaaacagaggtttcttgaaatgatcaatgggtagggctgaaaatgggcactggccctagccaggtgagtaggaaccgggcagggaagggcagagaggtgaggccctgaggtcagtcagacaggactgaccagggacaagccatgaccctcgaggacccaggggcacaggctcccagatgatagcccctctctgaatgagcacccaggcaacacagtccggggctgtgtgtagcaaacctgtcagcagctgcctcctgggacaaccacccccttacatgctatctatctaccagacaaatgaaagctcttcttaccccatctcccaggcaccccccagcaagggctctgaattctaaaaacagcaaaaacattcaaatggttacatatgaaatgctgtcctgcatctttctgtctcaaagatagcagctacccctcccccagtccccccccccatcccccaaacaatttctgtgccaagatgaagaggaggccccaggccatggggggctcctggccatgaggggctgttgcagcggcgccagggcacagggtgggcgagacacagcagaggtcctggcagcgcggcccaggtccccggcatctcctcccacgggtcgcagttacttattcagggagagtgactgcattcgttttcctgacaatgtggcatcgtcttttgctttcctttcctcttccttcttccgggcagcctcctcccgctgtttccggatgatggccagccgggccaggtcagccttggcttgctctgtcttcccggccaagtgcattttcatgtaacgctcttttgccttctgcttctcaatctcttctcgttctctcctcgaaagctcctttggcccgtccagatccagttgtgtgacctttttggttgtctgtgccacccggttggggttctcgatgtcgatgagcccttcaacgcctttgcgcttttgctggtagtcatcttcttcatcctcactctcatctgagtctagagatttcttctcctttttggggtcacctgcagccccatctccaccttctttttgctcctcttcttccctggccttctgcttctcagcctgcagctgcgcgtcgatctcctcagggcttgtatactgcctcgcccggcctttgtggcctccctttcttcctcctttaggcattgcggctccggcggctgcggcggcggcggcggcgcctcgaactgacacc

SEQ ID NO: 13779 - RNA, 8481 nt, Homo sapiens
  source 1..8481: mol_type = other RNA
gctgggattacaggcatgagccaccatgcccggccttaaaactgtatactttttgatatttttctttaagtaatcagtttaaaataatcaatgaatcattttaaaataaccaatctaattgaaccttgtccacagacttcattaaaatggtacattttatttggtcatcataaatttttttccaaaagccaattctcagacttgtacataacaccaagctttgaataacaaagctttgtgactgtttttttttttttcttagcatgcgcagggaattgccaacataccagggaagaacagggtgaaagttaatgagaaaaacagttatttgatttctactttccatatttgcttgataatgtttcctgaattgatgacatccctatcttggtcaagtctctgctttattctttcctagaacagaatatgcctaaatattgctatgcttgggactcatgaatgtttttacatttaaagattaataacttttccttaaaactttagagggtgaaaaaaatccacttaaacattgaaaagtctggctgggctcagtggctcatgcctgtaatcccagcactttgggaggccgagatgggtggatcacttgaggtcaggaccagcctggccaacacagtgaaaccctgtctctactaagaatacaaaaaaaaataggagtgatggtgtgtgcctgtagttccagctactcaggaggctgaggcaggagaatcacttgaacccgggaggtggacgttgcagtgagccagtttatagctttcagtcaagacatgtatattggttgaaatactgatacagttattctatagaaatttgttgcagcctgaaatgattttgatttttctctgttaaaatgactttctctgatacttaaatattttaaaataaaaaagcaatatctagaataatagtttaaaatacaaaataggtttctaaaatgaatgttatttgatttcatcatatattaacagattttagtaagttgtttttaaactagaggaattgaggcagagagaaatgaagtccttttactggaaattttcatctcttaatgtgttaattgattgatttttacacatttcattttaaacatggaaatgatgaaggttctaattgtaatgagtagttgtttttggattgttcaggtacactgcctcttttcttcagacactggggctcttttgtggtcactgagtattactgttttttcaagtcttcaagcacatcttgctttgtgattttggcccatgcattggggattttacctttacctgcaaattttttctgatatttttcttctagatttgatctgaagtgagagacaaaccatttccagtatagctggatggaggtatctggggtgatgctccacatggcataatcccctcctgcttgtcgatagttcttaaatgggaaattcctgccatccctcaaaaccaacaaacaatcacttgcaaccaaactagtacagcaatcaatgacaaaatcatctgtttcataccattcctccccattgacagcctgaggacggtggaagggaacactatggtctccttcatgtgtaggaattgtgtttgtacaaattgctccacagctgggacactgtttccagcagccacagagatgttcagagagcattttctcaattttagaaaccattgcttctataggcttacttgaataattctgttctattttcttcattgtgagatccaaagctgcactcatggcttctttaagaaattcagtatgttttatctcctggtgttcaatgcttatcaagtcccttcgtggaaagatcaagttgcaccccaggcaatcacagaataaatccaaccactcagaagcagtgctgcttttatctttagctactgatgtggattcatggatggcagagaggatggtattcttgatatcaattaagcttttttcaaaaaaagtcttcattttttcacctccattgtctgaacaatatcttttaatatgatttttgatgtaactcctaaaaaacgattttgaattatgaaggtattcccagtaattatcaaagttttcttcttctgccagagagaagagaatgtgtttctccaggttagtcctgtttccattgaacgcagggcaggtagctcgcatgtcccccgcaattttaaaggtcatgtcctcccatatagtagtggagactgcaggagtgagcttataccacagaacatcaacaaatgttttgatggaggttgctccttgacaggagatcttaaaactcgtgaagaaatcatctttcttactttctaggtagtttacaggatcatttgctctcttgaatgccctgtgcatttccttaaaattctctcttgctctttgaaataaacacacacataagtcaatgataaatgtatttgtaaatgtgtatctcttctgagtagaggcagatttcacttcttcttctattgtctttagaatctcatggaaataatttggattgtaaccacactgttgtttccacatgttgttaataattttattaaatcttgaaacaatgtagtcagtagtcatattaatgaactctttctcaaagactgttaatgtcattgggatatggttatatttcttattcaccttgatatgtttatcataattgatttgaaacttctctgcagaatttgtcagtagacccacgacattcgtcttgtttttgaaatactcccaaaggatgttttcagaatccaaatcaatgtcaggctctgtaacttgcgggagagttgtggatacatcacacacccactttttccaaagttgattgaatttctcatgtaactcttcctcactcaattctttgccctttacagttaaagccaacttccggcttttttccaataattctttttcataatctgtctttttcttattcagcctttcttgactttggtttttaaaactaatgagttcattggcttgtcttttgctatctgaaataagtttttctttaaggactattagcttattttcaaagtttgctttacattgaatcagtattttgctacatgggccttcattaaaatatttttcaagttcttgcttgacaacttcatatttttctgtaactagaacctcaaatgtgcttgcttcaagtgtctggatttttccattctgaatctggttgatcagctggttctgcaagcccagcacgtgactcctcagctcccaggtccagtggttatacatggtttccagtttgttcatggccatgacttcttgggtgttcctgaaactgaaaataaagttctcgttcatcaggcctctccacaaatcttgaactcgggattttacatctgatatcttcatgatgtttcccctggattcctgtgtggcagtcataagaattctacttttcagttgctgtacattgtggctgtagcgaggattgggaggggccattggggggttgccatcccagaggtgagcaaagtagtagacgtgagtattgacatcaaacctaatgacatcactgaagcaggttacgtctaagcactgttcttgttcagcagctattgctgccatttcatctagtttctgctctagccgtcttcgtccatccatagtttggtccgtagctgtagcttcccccacattctgatggacaaagaggcaacttggaaagatttttacttgtttcattctcagaaaggcttggacaactatttgtaggatatcttgcatctctgatggattctccccaaaaatattgatcagagtcaagtttgcaagtccaatgacaaaagttaccaactcattgtccctatccttggatttgttgctgtgttctggtgcccgaagtccttctgtgtccacagcaagcacaaagtcaaagccaagttcctccgtgaatgtctcctccaccttgaggagctgcatataggccccttgggtacatttgcctgcactaacagtgaactgaagcccaaaaagggcattcagcacggtggatttccctgagctctgcaagccaaggatagaaagaacaaatagccgtttgtctccaagtttctcagagaccttgtcaaaaacagctgccacccatgttagaggtacatatgctgcatccccatccatcagctcaatgggaacaccagatatcatcaggtctgcggcaatttggggaagcgagaaaaaaatcttttttatggaggaagcttcttccagagcttcataaatctgaccaacttctctgataagttgctcaattcccaaagtacagtcactaatctctgtggaaatggcttctatctcactttgcaggcatatcagggagtgactattaggtgccttttgctttactgtttgaaccagtgaccaccaatatttttgcttctcatgcagttcttccaagtgtcctgcagtcagtttgtccaaaaatacactcagccactgcaagaagtacagtttggtgtgaatttctgaatgctcttggagaaactgaaggacagattgcattaaatcattgagaggaagggctctggccaactgttcatgccgtattatttgtttatctgtctcaatctcactcttgtgttgttcaatgctctgatttcccttttctctaagatgatagagttctttgtccttcttacaccagtggtgccacagttgtccctgaaggggtagtaatttttccttaatctgagataatttcattttccccaggaaggccattagagcctgtgccttttctttggcttccttgcagtctctctggtcttcatcgataagaaatccttgctggtgagcaatctgggaacagtcctccaagctgagagcagtatctgagagttctagcaaatgtctgattgtagttgtgagttcctctgttaattctgcctcatttctattcttgatacccattctcattctttggccagaaatattggtcatggttgcttctttgtcatcgagcaagcagatcaatggccttgatgactgccacaagttacggacaatttttcggtttccttcattgtcatcggaggctgacatgaggaccacaatgacagtagacacctccttcaggaagctgagctgctgctcatgttcttttgcatctccatgaagattggtgaaggtcacacagttgtcaaatctgtcctcatcttcccctcctggacagaaccaacagatctctaccatgccccccatcaagaggcagtctttcctgcttcctgtgcagtgtcggtgaaaaaacacatcatgtttccgtttactgagaagacagttcataatctgagatttagaagcagagaggccatttccaactcttacgaaggacacaattgaggtagagacacagcacatctgctgattcttataatagttcttcccttttggtgatttccttgcttcctgccaacttcttgtaatttgacggagagaccagagagagaattcaatctgagaagtacagggattaggcaccaaaagggggagggcaaactgacaagtggaaagtttggccaaaatatattgtctggcaaaattatctgcacagtgaaaaattgtcatctgaatatccactgggtgaatgtgggggctaggctcagtggatgaagatttagtgggactatcactgtcttcaaaaaagttttcatatgggtcaaaagcctcatcttcctgatctgaagcatttggatgtacttggtgttctgtgtttctatcatctttgaagactaggtatctcagctcataatccatcatcagtagtttctgcaggaaatagaagggaagctcctgttcagagctgggctgggtgttatacacagacgtcttatagatgagatggaaattagctttgctcaattttttggggtagtaatgttctagacctagatgctggagtaagtctaggaaggctccattttttatcatctcccatttgttattttcattgtcatgtggttcatggggctgtttctttccatagaagagactttgcttgctcacctcttccatttgcaaagaagagatggtgacttcttcataatccccattaatgagcaatctcaagtctttctctaggttttcccaatcgtgatctgctccaggtttggtgaggacatgtgcaacttctttggacaatgattgtcccatgtgatgtctcattaatgacatgcgttgtgttttctcttctgaagaaatagctgtgtctccaactgtggctgtcagacctgtgagaaccaggaatgcctgagccctatagctgcaaatattcttaagctcctggtatttattttgggcggtttgcatttcatccagtaggaagcttaactcatcacaccccaagagactctgaaaagtattgttgatcacatgatatcctgcagcagctgcaatggaaagtagcaagagttgtgtgtctgtctgctctgttttttggagataattcaagaagcagctgagagccaagctgacctcataagtggactttctttgagcttcctccactgtttctggggactcagatttgacctttacttccatgaggttattctgggtttcttttaagatctcaattaattgagaaaattgggaaatattcacctgctcctgctctgaatctgactggaagatccactgcatgatgaagtgagcctgaggaaagtttgtcactctgtagatgtgaggatccagaaggctgcgcaaatgagatttaatacatttagttttataaatggaagactttttgcaaaagttgatggtgtttactagaaaattctgcagactctaatctgtgagacatatattaatccaagtgtcataactttttagtttttgactcaacattttcatgaaatttatcagttttttaagttgctcttcaggatcagatacctcccaagattttacatcctctagaaaaaccctggcctccttcccagcactcagtaactcttccccattctggatctgggcagtgatgctagtcagagcagtgtagctgtctttcaggaagttagccacctgaagaggatccttaaaattgcttctgtggctagagaggataatgtcccaaactggcaccaactgaagcccgcggtcaatgacacaccaggtttgattgctggcaatgaggccagctttccactggacaaggccatctgcttctggtgggccacctgtttgggccacagataattggaccttggtttggaggttttgggaagttttggtctgagtggctgtcttcgaatgagagtctgaaacattcacacctgcagcaactttcactccaaagccactgtagctgtcccttatgaaaatgtccagggcctctgcagactgctgcctcacttctgccaactgctccgtgcaataaccctctgaaatggctttccaccagtagattcctcccaggtgcagagggccttggttaacatgagagccaaacctgtggaagaagtttatgatcctgtgcctcagcaaggagaacctgtctgggtttgttgtctgactcagaagctcttcaatgcatttcaattcctggacagcaggcttggataactggagctgatcaatgggaaagtggcaggaggccagggggatatagctgaacttggttgagcagaaataagaattctcagaacttgattgttgggtttccttggattctggatgtttgctgtgatccaaaccagcttctagactaaacccccaatttccgtccttggctgaagtagttaaacgaaagcccagcttctctaccatctgggtaaacatgaattcagcctgaggagatgtgaattcctttgttttcatttgtgttccttgctgaggacccaaaagtaagaactctttggggacactgagcaactcctctctcttctctgtcaggcccctttggtggctggctttgtaaattccctggagggccagccctccagatgcccatctcaccacatctctatctggaaggttttgcctgtggcacagtgtccacttcatgaggttgagttgtctctgcaggttttccatgagttcccttagaggctcttcaggggatggccagtactcttcagggatgtccattgcttgcctcagctctgcttctcttgtcctcactgcctcttcctgtctctgcttcccttctgtcagcaagtccctcagctcctgcagtgcctgttctgcctgcttctgctttctctttgccctctccacctgagactcctgtaacgctgaaagactttttgagtgtgacagattaagcagctttctcccatggatgttgtgtctgggatttcagcttcttgaggttgtttttgtctaggtgttgtaaggcctgggcacaggtcacacccaggtgttcctgcagcttgggtaaccagtactcaacatccaggcccacttctctcagcatctcttggaggtcttgcctccttttgcctctgagcagagggtcatcaggggtgtgctctcctgtggcca

SEQ ID NO: 13780 - RNA, 1143 nt, Homo sapiens
  source 1..1143: mol_type = other RNA
gctgggattacaggcatgagccaccatgcccggccttcttccttctagtctgacaggacgatgagctaaactgaacatctgcatggcaatagcaaagtcttccaagtgggttgtaaaatggcaaaatgacttgaattcatccaaactaatgctctctcctgctgacaacttctctctcacatttttccaataaatatctttattttcagtgttagtgaaaaaaagtagccactctgcaaagtcttcttttctcatgaaactcaaacctttagaaaactgaaggaattccatttcttgaatctctgtttgtaaattttccataaatcttcgaaattctttataatgaagttttctttgtcctctttttccaaagaaacgcatctgaagagttgtgttaatttcaggttctttcactattgcttcctgatatccagtttcattagttttcactgtcatcaagtcatcttgtttacttatgatcttctgcagcttaaaaaattcccttttttcaatcatctcattaccatctgtatccagcattttaaaagcaacatgaaatccagaatggggtttagtgaggattgtaagcaagaaaagatactcggtatatgaaattagccctttatcgccaaggtctctgaaaaaagttgatccacagccagctgtttggatccctgacagtgtatcctcgatgtccttttttgtcagcttcttgactgaagttttacgttccatttgctcaaacatcactgagaagaggaagtctcgtggtgtcatataatattctccttcatgttcgagtgaagaaaactgcatgaagcgctgcttacgaagagacggtttcccaatatatattattccatgttcaacatttttctgtgcggagactgtaaaactgccatcccgcgccgcaacactgacgcggctgtggtgccaggccgctcctgctcctgccagggccgcgccggccactgccgctgccaaggggccgggactccgcacagcctgtcggctgacagcgagcccccgtcgcagttttccgccccaggccgccacccgcgcgcagctacccgcagccgccgccatctttgcggaagcgcagctaggcggcgcttctctcccggcgccgccgcctaccgcttg

SEQ ID NO: 13781 - RNA, 3704 nt, Homo sapiens
  source 1..3704: mol_type = other RNA
gctgggattacaggcatgagccaccatgcccggccttttcttcttctatttttatttttttaaatacaatccacggtcctggactagatttcaggacttttcaagagaagctggaaatccattttgcctgagaaatgtgttgttgttgctatgccaaattaaatgcacacatgactggatttgttgtttctgcatgttgtaatagttctgagcatgagttcgggagtctggggtttgaattttggcggtaccactcatccattctgcataattgagggtcccagtttcctcgtctctaaaatggaattctacctcataaggttgtgtgggtttttttttttttgagatagagtctcgctgtcgcccaggcagcagtgcagtgctgtgatcttggctcactgcaacctccgccttccaggttcaaacaattctcttttctcagcctcctgaagagctgggactacaggtgcacaccactacacctggctaatttttctatttttagtagagatggggtttcaccatattggtcaggctggtctcgaactcctgaccccaggtgacccacctgccttggcctcccaaagtgctgagattacaggcgtgagccaccatgcccggccctcaagatttttatgaggaccacatgaaatgctgaaagcacttagtagtatgtccaggagcagggtcttgctctgtcatctagacttgaatgcagcgagtggcatcgtcatagctcactgcaggctcaatctctcagcctcaagcaatccttgcccctcagcctcctaagtagctgggactacacgtccagctaatttttgtatttttgtaaagatggggcctcactatgttgccttggctggtcttgaactcctagtttcaagttatcctctcaccttggcctcccgaagtgttgggattataggcgtgagccactgcaactggccaggacagtgattgattgattgattgattggtttgagacagagtctcactctgtcgtccaggatggagtgcagtggcacgatctcagctcactgtaacctccacctcccgggttcaagcaattctgctgcctcagcctctcgagtaggtgggattacaggcacattccaccatgcccggctaatttttgtatttttaggagagacagggtttcaccatactggccattgctggtctcgaactcttgacttcatgatccgcccgcctaggcctcccaaagtgctgggattgacagtggcatttaaatagagaccttttagaaaagtgggaaagtagaaaaataaataataaatacataaatagagacctgtaaatgatgaacagtgaacttggtggagaagtgagatgggcatggggaggatagccctcaagcagagggaacagggtagaaatcaatcatgcaacaccaaattcaagcagtgaggatagaggggacagccaatcctctagggagggctaaggatttcctgactgataaagcctgagcggcaaagaagcctcctatccagccttgggcaagtctctgccaagctgggacttcacactacactggccagccattgacttccctgatagaaaaaccacaaccaacaagtcctcgctggggctggtctgccaaacacagaagacagagggaaggggagggggctgtcttggggtcagaagtgagcaggttttccaggggagaaggaagattgagaagaggggtatggctgctggctcacacctataatcccaacacttagggaggccaaggcgggaggcacacttgtggccaggagttcgagaccagcctgggcaacatagcgagacttcgtctgaacaaaaaaaaattatagtttaaaaattagctgggtgtagtggcgcgtgcctgaagtcccaggtattcacaaggctgagggaggaggatcgcttaagcccaggaggtcgaggctgcagcaaactatgatcctgcaactgcactccaacccaagtgacagagcaagaccttaaaacacacacaaaaaaaaccaaaaaacggcagaaagatgagaagccgttccatttgcataggcagttgaagtgtctaggcagaggcctccaaggctgactggatatcaggcaggggatgaggctggacagcctgcaatgcctccaactccaggttgcggaaatcgtgtttgtagtacctcagtcgaatggagattgagcgccccctgggagcagtgctcggtaacagacgctggaggaccccgatgaggaggggcgggggtcggttcaatctgggaggagcctgcgggtcagttttcttctcacaggagcgaactctgtccggcatcatggattcctgggctcccagaacggctgggctggaagggaccttagaaagggatctaccaccgcgtgccccgtgccagagttgggcactttggtgacaagaacattggcttgtttaacactcacaactgtgcttcgaggtggggatcattatccccattgtccccattttgcagatgagaaaaagcaaggtttggtggcttcccggggcggggcggggattcgctgtgactccaggtccttttccccggagcccgcacgtcttgtaagacactgattcccggaggtctgaggagcaggaatcgagtgggaggtgcccaggctttctagggaacaagagtgtgaatgcactctcgacgagaaccacgcccccctgttcgacaagactgattcctgctgccttcctttaagggccctcccctgaaacgcgaagtcctcgccccatggagaggcggacattctttattcccggatcgcccgacgtttttctcccccacccgcactgatccccactggtgacataaatccttcccctccactcgcgagtgaaagcttgggactacatttcccgccaggctgttcagaagccggtggcggagagaggagaaaagagtctttccgtttccgtcgcctcgcaatttggcgtgtccgccgggattcacatttcaacagcgacgtcctttctctgttggactcggcaaggaactacatttcccagcaggcaccggcgcagaggtcgaggggcgaggtcgccatctttttcgtagtcctctccctcatttccgcagggaagaggccagacgcctggactacacatcccatgtcgcagtcgccccggccctgcagccgccatctttgccggtggccccgccccatccccttccattgtctcgacttgagatgatagacgggagccgggagactgcaactcccgtcaggccgtgcgccactggtgggggggatttcgagaccacaggcgggcgaggtgcccaaggtggtggaaagcggagaccgggagaggctaggtagcctgccatctttacggtagtctcctcgtcctcctggttccgccattcttaaggaacactggaaggctataaaactactaatcccatcgcacctcgtaagatcgactactagtcaggtgtatgtccctcttccgccatcttgcttgtagtcctctttccttttcacctttccattgttcctgacgagtagaaatggcagcgggaaggcagcagatggactgcgactcccgtcaggtaccacacacgcggagggttgtggacaggagggcgtgtgagtgcctgggaaggaggtcgggtcgggggagaaggccatcttgtttgtagtcatcgttccctctccttctcgatgtt

SEQ ID NO: 13782 - RNA, 3265 nt, Homo sapiens
  source 1..3265: mol_type = other RNA
gctgggattacaggcatgagccaccatgcccggctagtttttttttttttttttgtattttcagtagagatggggtttctccctgttggtcaggctggtctcgaactcccaacctcaggtgacccacccaccttggcctcccaaagtgctggaattataggcgtgagccactgtgcccggcctttgccaggtatcttgactagaggaagatagtgttctgggtgggagactcaagaggtctggttactgaagatacagatctcacttaaagtaagtaaattgacatctggtttccaaatcaatctattatgaaattggcccatgtcactttcatttggcctgatcaagtttttactgagaactgaattgggcacagtggctcacacctgtaatcccagcaccttaggaggctaaggcgggaggatcacttgagtccaggagtttgaaaacagcctgggcaacataacaaagtcccatctccacaaaaaatacaaacattagcccaggaagctgaagcaggaggatcatttgagcccaggaggtcgaggcagcagtgagctatgatcgtgccactgcactccagcctggatggcagagcaagaccctgtctcaaaaaaaaaaaaaaaaaaaatttgagaacattggacattcagtatctctcccctctcttgggcatcatgtttaggttctgtctctagagcacatctcagagcctgctacaggtaaacaggccagaagttaaatgcatgaaacaaattaaatgcatgaaacattcaagcacattcttattggtgtaattaaaataaaaaagtaaatgcatgaaacagaagctgtttacccacagcagaggaggggcagaaatcatatccagtgtgccatatcattactgcctgccagcatttccttaggctatttcatttatttactttttttgagatggagtctcgctctgactcccaggctggagtgcagtggcatgatctccactcactgcaacctccacctcccaggttcaaccaattttcctgcctcagcctcccaagtagctgggattacaggtgccagccaccatgactgcctaatttgtgtatttttagtgagagacagggtttcactacgttggccaggctggtctcaaactcctgacctcgagtgatccacccgcctcggcttcccaaagtgctgggattacaggcgtgagccaccatgcccaccttcctttggttattgagatggacaaagagttacccagtaagttaagagcagctagtttttaatgaatcttagcccagaatacaaagcagggtgtagcagttgccttaatggtgatataattgtaaacaatagctttttcttcccctataaactcgagttataggaagcgtttcagagagaggataacacatttgaatctattttttaaaaatcatcctgaaagctagcagtattgttgtcgtttaaaaggttcctcatatactcttaccctcagccaacccaccatgtttatcaattcaaattctagaactttcttgacccaagagattttgtaggaaaaatttctcttttcagatattcagcacgcaaggatcatttttcttggttttgttgctgatcttgctgaactttccatcaatggctgagggaggaagcttgcatgattcttatgagttcttctgaggcactttgactgtgacagttttcacttcagtgtatgcctgcagcccgtactcgcccaactcccggccactccccgacatcttgtagccaccaaagggtgactgggctccaaacacatcatagcagttgacccacacagtgcccgcctggagggcctgggacaggtaattggccttgtccaaatcctttgtgaagacagctgcggccagcccgtacgtggaattgttggctctcccaacaacctcctctatggtcttgaacttcaggatctgcatcactggcccgaagatctcctccttggcgatggtcatgccatcctgcacatctccaaacacagtgggctggatgaagtaaccacggtcagcagcaatgcccccaccacacagcagcttcgccccctcttgcttccccgtgttgatgtagccgaggatcttcttaaactgagtttcatccacctgcggcccctgctcggtcttgctatcaaaggggttcccgaccacccgagacttggcccgggcaacgctccgctccacaaactcatcatagatgtcctcctgcacgaaggtccgggagccggcacagcagcactggccctggttgaagaacagggcgaagtgggcctgttccacggcccaatccatatcggcatctgacatgatgatgttggggctcttcccccccagctccaaggtcactctcttgaggttgctgctcccagcagcaacctggattacgcggccaatctcagtggagcctgtgaatgccactttgtccacatcctcatgggaggcaatggcggccccagccgtggggccaaatccaggcacaatgttgaccacaccagggggaaagccagcctccttgatcaggttggccacatagagggcggtgaggggtgtctgctcagctaccttcatcacaaccacgtttccagttgccaaggctgggcccagcttccatgcttgcatcaggagcgggaaattccacggaatgatctgcccgcacacccccacaggttcatggcgtgtgtagctgaagaagtctccgtcaatggggatggttttcccgtggtacttatcagcccagccggcataataccggagacatttgaggaccatgtccaaatccaccaggtaggagatgacatagggcttgccattgtccagggtctccaaggccgccaggtaggtccggtcccgctcgatcagatcggccaggcggttcagcagccggcccctgtgtgatgcgtccatgcggcgccaaggtgagcccagctggaaggcggcccgggcggccttcactgccttgtccacatcttccttgtccccttcagctacctgacagatgacctctccagtggacggattgacggtggggaatgttttcctgctgacggcatcgtgccattcattgtttatgaaaatctggttgcagaagacctcgggctgctggttgggggcaggcacggcctgggtggcggcggctgacaagaggcggcggcccaggcggggcccgaagcgggcggcagcgcgcaacatcgcagcgggctagcggacagcgagcggaccgagagcagagctagggtctc

SEQ ID NO: 13783 - RNA, 3124 nt, Homo sapiens
  source 1..3124: mol_type = other RNA
gctgggattacaggcatgagccaccatgcccggctagtttttttttttttttttgtattttcagtagagatggggtttctccctgttggtcaggctggtctcgaactcccaacctcaggtgacccacccaccttggcctcccaaagtgctggaattataggcgtgagccactgtgcccggcctttgccaggtatcttgactagaggaagatagtgttctgggtgggagactcaagaggtctggttactgaagatacagatctcacttaaagtaagtaaattgacatctggtttccaaatcaatctattatgaaattggcccatgtcactttcatttggcctgatcaagtttttactgagaactgaattgggcacagtggctcacacctgtaatcccagcaccttaggaggctaaggcgggaggatcacttgagtccaggagtttgaaaacagcctgggcaacataacaaagtcccatctccacaaaaaatacaaacattagcccaggaagctgaagcaggaggatcatttgagcccaggaggtcgaggcagcagtgagctatgatcgtgccactgcactccagcctggatggcagagcaagaccctgtctcaaaaaaaaaaaaaaaaaaaatttgagaacattggacattcagtatctctcccctctcttgggcatcatgtttaggttctgtctctagagcacatctcagagcctgctacaggtaaacaggccagaagttaaatgcatgaaacaaattaaatgcatgaaacattcaagcacattcttattggtgtaattaaaataaaaaagtaaatgcatgaaacagaagctgtttacccacagcagaggaggggcagaaatcatatccagtgtgccatatcattactgcctgccagcatttccttaggctatttcatttatttactttttttgagatggagtctcgctctgactcccaggctggagtgcagtggcatgatctccactcactgcaacctccacctcccaggttcaaccaattttcctgcctcagcctcccaagtagctgggattacaggtgccagccaccatgactgcctaatttgtgtatttttagtgagagacagggtttcactacgttggccaggctggtctcaaactcctgacctcgagtgatccacccgcctcggcttcccaaagtgctgggattacaggcgtgagccaccatgcccaccttcctttggttattgagatggacaaagagttacccagtaagttaagagcagctagtttttaatgaatcttagcccagaatacaaagcagggtgtagcagttgccttaatggtgatataattgtaaacaatagctttttcttcccctataaactcgagttataggaagcgtttcagagagaggataacacatttgaatctattttttaaaaatcatcctgaaagctagcagtattgttgtcgtttaaaaggttcctcatatactcttaccctcagccaacccaccatgtttatcaattcaaattctagaactttcttgacccaagagattttgtaggaaaaatttctcttttcagatattcagcacgcaaggatcatttttcttggttttgttgctgatcttgctgaactttccatcaatggctgagggaggaagcttgcatgattcttatgagttcttctgaggcactttgactgtgacagttttcacttcagtgtatgcctgcagcccgtactcgcccaactcccggccactccccgacatcttgtagccaccaaagggtgactgggctccaaacacatcatagcagttgacccacacagtgcccgcctggagggcctgggacaggtaattggccttgtccaaatcctttgtgaagacagctgcggccagcccgtacgtggaattgttggctctcccaacaacctcctctatggtcttgaacttcaggatctgcatcactggcccgaagatctcctccttggcgatggtcatgccatcctgcacatctccaaacacagtgggctggatgaagtaaccacggtcagcagcaatgcccccaccacacagcagcttcgccccctcttgcttccccgtgttgatgtagccgaggatcttcttaaactgagtttcatccacctgcggcccctgctcggtcttgctatcaaaggggttcccgaccacccgagacttggcccgggcaacgctccgctccacaaactcatcatagatgtcctcctgcacgaaggtccgggagccggcacagcagcactggccctggttgaagaacagggcgaagtgggcctgttccacggcccaatccatatcggcatctgacatgatgatgttggggctcttcccccccagctccaaggtcactctcttgaggttgctgctcccagcagcaacctggattacgcggccaatctcagtggagcctgtgaatgccactttgtccacatcctcatgggaggcaatggcggccccagccgtggggccaaatccaggcacaatgttgaccacaccagggggaaagccagcctccttgatcaggttggccacatagagggcggtgaggggtgtctgctcagctaccttcatcacaaccacgtttccagttgccaaggctgggcccagcttccatgcttgcatcaggagcgggaaattccacggaatgatctgcccgcacacccccacaggttcatggcgtgtgtagctgaagaagtctccgtcaatggggatggttttcccgtggtacttatcagcccagccggcataataccggagacatttgaggaccatgtccaaatccaccaggtaggagatgacatagggcttgccattgtccagggtctccaaggccttgtccccttcagctacctgacagatgacctctccagtggacggattgacggtggggaatgttttcctgctgacggcatcgtgccattcattgtttatgaaaatctggttgcagaagacctcgggctgctggttgggggcaggcacggcctgggtggcggcggctgacaagaggcggcggcccaggcggggcccgaagcgggcggcagcgcgcaacatcgcagcgggctagcggacagcgagcggaccgagagcagagctagggtctc

SEQ ID NO: 13784 - RNA, 3727 nt, Homo sapiens
  source 1..3727: mol_type = other RNA
gctgggattacaggcatgagccaccatgcccggcttgtatctgtattaaaacttgactctgccactcttggcaatatgatcttggatgaattactttttcttcctgggacttgatttctgactctttaatcagagtaacactgtctacttcaggagatgtactgaggattaagtgaaatatcctatgccaagctcttagaacaatattgggtacatagtgaacacttagtaagtgatgactattgttgctattgctacgattatttattttaataatcttaacatgtagcttcatgtctggaacattatgtgctcagaaaatattactttcacccttcttcagtatctgtttagttgaactggatctgtagaggagaatattttggatattatcaatctgaactaggctaagtggttgccatttgcctaattttatttaattttctacgattttcttcctcccttccttcctgcttgtttgcctgcctgtctcccttcctttcttctttctttcattgtccttcctaccttctttattcttctctgtctcttccttttatttctcaaccttttttttcccaagcagatattattttaaatttccgaacaacttatgtcagcaagtctggccaagttatctttgaagcaagatcaatttgcatccactatgtcacaacctggttcatcattgatttaatcgctgccctgccttttgatcttctgtatgctttcaacgtcacagtggtgagtaaagagctccccgccacatggcctttaaggttgatttatttatcgcatgttcaggttttaaatgcttgtggcgatttatgcttccagggttttgtgccttcttcaataaagatgccctgatgcccagtgatatgcaggccagattcttcagttgatgaagttacttccttttgacattcatattagctgttcatgcttttttcaataccctttggctggagcaagcgtatccattgcagatgcctaaaagtgtatctgtatcatgcggggtagggtgggaaggccaagaatctagaatgggaaaaaagggattaagtcagacatcattttcaaattttcattgacaattttaatcctaaatctcctgatcctcgttggataaaacctcataaatgctgattgatttgaacggctctctagttattaactacttagcatttacaagccttttgtaagaaaaaaaaatgaccaggcttatgatgttgtaggctgattacttcagtaactgcatcggttttcctaaagaaggttgaatttactaaccctactttttcagggtttacataaagaattataaaaacttttaaagctaacccttacttgtagattcgcattcttaagaatgcatgagataaagaaaagaggaaaaaatctaaaatgaagttttccagccattaaagtggacactagtgaaggactcctggatttatttttttaaaacataaaccagtaccttaagccttaatgtgcactggaatgaaccaaggatctcctttaatataaattctaattcaggaagtctgaggtggagtcaagaccctccttttttaaacaaactccacagtgatgctggtgtcactggtcctgcacaccggactgtgggtggcaaggtttttaaaatgtcttgagacttttgaggaagttaatactcccagttgtaaacaacactaaccagtaacaattcagtcctttctatccttttccaccgtcctatactttttcaatccccaacacatctgcaaatttatttggacatagtttatttctgatggacaaaggaggtctatctaaaagcagttaacctcaatactgaagtagtacaacacagtacttaaaatgtcatcacaaacaatttatattactgttagttccagaagacgcaaatcaaataccatccattttaaaagttttgtcaatgctctattctattttcataagggcttctagaaaacagaaaatatttccacgttttagaagtaagattttactcttttgtcgtaaggagcaaatggtatattttaaagactcaatttttttatattttaagtatagcaataaactttgcttcttataaaaatagaggaagtaaagtatatatagcaatgtccaattatgaagttgcattatctctgcagtctgatctcgtatttaaagattattggggcatttagatagtaagaaatacaaaaatttgcatttaattgcataatattctcagtcctttgaaagggaatttctgggtttcaggtagcagacagggagttaatatgatttcaagttgccacggttgcttaagaggagaaaatacttatacctagaaaggaatgaacctacaatatactcagtatctttgcaccacagtttccaaatgtgttcacacttcctaccaaacactccaagcaacaaagattctgttatcatgtaagtttgagaaatgtagcacactgcatccctgttcgtaaagactgagaaggtatattagcagcatataataagctcagagaaattctgaagaaattgattaaactttatttaaaagaaatgttgcataaatttattttctatcataatctttttcttttttgtacatattgttaatactctattaacatcctatcctatgaatttgaagttttaaaaacacaccttaggaaaagttactaaaaccaatatcataataggaagaataatcatggttttaatcttttaaaaatataggacatcacatgtatcatcctacagtaaatctacaaaaatagagagcaagattattctcgctacaaaatggagataaaaatgcctacttagaaaatcactggtgagcgtaaataagagtatatgtgaaagcagtttgcaaattgaaaagtgctatagaattatgatgtgttatttttgggtcatagttaacagtatacacacatatacatacatgtgtatatgtatatttatgcatgtataagaaagaaagacaggaatgtgtatatgctataccacaaattcctgtcttcgtgttctccacgatactgatcctagcatggatgtagagaggacatgcacaatacatgtatttgagtgaatggatgcaggaataagtgggtgaacaacaaatagggattctgtaccttattactaggtcaccctttagcttaaacgagaaagacattctgaaatcagtcttccttcagtgtttggaagttatgcttgttccgtacttccttatagtatctcatcatttatactgtacgattataggccacattctcgttagtcatttggttaaaactgatttgcctaaaatatagacaataaagttataggaaaccaaaagtcaggattctatttctattcaatagtctattcttttggatattttggctacccaaatactgaagtcccttagtattcagattacacttgaggagaaactgttttggttttctctcaaaagatcttataatacctgacaattattaatataagttttattaagcatttataaatatcacaaattaatccacttggggtttggttttctgatttataaaacagtatccaagtgtaccttgcccctacattgtccttgctcttttttgaaaatctttgaccttttatacgataattaacttgcaatctgtactctacatagtcctcacatctactgacaatctcatacaaacaattactcactttcttctgt

SEQ ID NO: 13785 - RNA, 6095 nt, Homo sapiens
  source 1..6095: mol_type = other RNA
gctgggattacaggcatgagccaccatgcccgggtagaagtctctttctttaagacccttcatgagcatgagggctgcctgacaaagtaggcaggactgtgattctttaaagacatgaaattaactccatagtcacccagttttatgcctgggggcactctccaaaactggacacagagagttaagctcaaaaagaacagtggtcttaatgggcacagaaagatcacaatttagggctgttgagaaaactgaattgtgatgcagggtacagaagtggaaactccactgaaaaagagctccagaaatctgcacgaggtgcccaagaacagaactttctgcaacttgtatctgtgacatctaatgtggtagccaccagtaccatgtgctactaagcacttgaaatgtggcaaatgcaagtaagaaacaatattttaaattaattttaaatagctacaacttgtgactactgtatcagccattatagccctagaagttggctgaacagttggctgaacagtaggctgcaaatgtgcagagcaaaattctgagacatgacagaagcctatgagctgaacagagtacagaggtggcaaaaatcagacgtggctctgaccaagcagaatggagagcctttgctgaaccatatgggctttcagtttagacaaagaaaggctacacttaagctgggcacagtggctcacacctgtaatcccaacactttgggaggctgaggtgggtggatcaccctgaggtcaggaattcgagacagccctggccaacatggtgaaaatctgtctctactaaaaacacaaaaactagccaggcgtggtggcaagcaactgtaatcccagctactcaggaggctgacgcaggagaattgcttgaacccgggaggtggaggttgcagtgagccgagatcacaccatcgcactccagcccaggcaacaagagtgaaactctgcctcaaaaaaaaaaaaaaagaaaagaaaagaaaaaagaaaataaagaaaaaatattgctaaagctttggaaaagaactgttggaatctgtggcctccttgagtgaggtctcacccacccctaggttgattggtaaaaactacagttttgtctggctgtagctaactgaaaaactagcaactttgccgtaagaggagtcttgatttacagcagaggtataaacctacaactttgtaagtcaaaagtaaaaaaatcacttaggaatggacaaggagtatctgtagttgctaaccaaaggttacagtcctagttcttgaagagcaacagagcagccagacatttaacaaggtcctggaaacagaagggcagaaaagggtaacatgagctctccaaacatctttggcaaactgaaatgatgcatgcacaggggagactcaagagagcatggcaaatgtaaaaaccaaggggaatttgggaactgcctcctacaatgaatgcatcccccatcccacacagaacaaccaacagtgggtggaaggcttatagactcaagtgtttgatcttaacctttgtccaaatgattggctgactgctaagctatgcagacacaggaactacccctagcaagcaagaataaatattgaaataaagaacttaaaaactgagcacagacagcaataacttcacatcatatataagatagattccacaatttgagtccagtcaaaatgctaaatttaaaacaatacaaatcccttagatataaaacaaaattgagttgctacaatatgctacctaaaatgtccagctgtcaaccaaaaattattagacatgtaaaaacatatgaaagtgaaatatactaaaggaaaaaaagcattcagtgaaaactaaatctgtatgggcccagatacttgattagtcaagccttcaataagacttcataacaaatatattcaaagaaataaaagtaaaaaaaaaattaaaaatgactcaataaaagagaaatcacaatagaaaattataaagtataaaaaaagagccatcacacttcattcttcctaagtcctacaccagagttgctttaaatgtgtgtatttaatggttaaataagacctgaaaagggagttggcctaaaaatatttttaccgtaaaacatcaatttcttcagagttaatgagaattatatgctaaccataccaaaaaccttgattagaatttttagcttagatgtattgattgatattaaaaagggaaagttgaggccacatacagaaagcaatggcgaaggacactgcctccaacagaaaatatgaaccaaaaagcataatggaaaaacatttacatgtaatatactaaatagatgtcatgccaacacagacacacaaggtgagaataccatgtgataatgcaagtagattgaaatgctaccggtgcaagccaaggaatgccagaaattgccagtaaaccaccagaagttaggaataaggaaggattctctcccttacaggttttcaaagacatcacggccttgacaacaccttgatttcagacttctagcctctagaactgagataataaatttctgttgctttaagtcactcattttgtggtattttgttacagcagttctaggaaattaatacaaacatgccttttaccacagttctctcccattggattatttaataataaatgatttaaaattagtatttggaaaagatgttttttaatgagtagacatattaatcaggtctcttttgacacagaaatgttctatatttcattttcatattcttgtcaaattataaaaataatatcataaatatggacatcgctacaagctattatgtacagtcactgaaaaatcagaaaaaacatgtgagttagaaatgtttatcaaatacaagtctacagaaaactgaataaaatttttattttaaaacatcacaagtaattacaaagacaaatattccaactatacaaactgtttttcacatatacatatatacatacatatatttaaggttggttgatctttcatctttttatctgagtaaaaagaagaacactttcctcattccggagatttttgatgttataatagttacctgaaggaacatagaacgaatccccagtacttaatatataaggtgtttcatgtaaagtacacaaaaggtcaccaaagttaacataaaaaaccaatatatcctggccaacatgctgctttcccttttcttcttgtggtcctaatatcaatttcccagtagaaaaaaagggtgtatccaatgtcttgtataccttcaactcaccatgcttaacaaaaaattgatatgtatcttgtggccttacaagatccatgagaataatctctcttgtttctgggtcctttaccctcgttggctgcaaaggatctccaagaggtatacctagatttaccattaagttagtctctatggtattatttctgaagtttttggaagtaaatttcatattttgcaaagagcttcttctcaaagtactcctatttaaaataaaatctaaaagttactttcagaaataagttcatacttctttcatcgttatcaagacagatccttttcttattagattttttgttgacttttccaatattttcttttgccttccttttagacgatattgtgtctggagatagtactccactaatcacgaatcctcctgatggccttccttgataatctattcgctctcctcgccagtactccaaaggtttcaaacgtgttctcttggtcctgcgaacatttggtgtgttggagggcaatactagtttgtgatggattctgttctttggtatcactttagattgttttgagtcatctgaacttccatgaacttcctcatcatccacatcattctttccagacattaaataattattattgagcctggaaggtccactttcctctaaaactgaagtcttatgctctccagaatccaagtttgactctgttggtatattacatgtatatccactggtctgaggctttaggggaacattctgtgcagtcataatgttatcttcattctttgagcttcttgtagatctagaacaatcaagatttttcttcttagccaagtctgcctcatcactttccaatggctcactcagcgaacatctggaaatttcatcatgaccaacgatacctccagaaccttcagcatttaaaaacttctgtactctttggttgcctttagttgctgtcttctgccttttaagtggaatagtttttttcctaatattcttagatgactgatttgttttcttagtagattttcggctactattgtgatgcattggtaattcatttcttactgaagaattgctataaacaggactctcctctgattttaccacccaccaatcagatggacgcctggaaattcttcgacttttcgtgacagttgaagtcacttcttcaggtacaagtttgttcttggactcactggaaaagcgcttctttttagattcttccttatcttttctagtgctacttttcttgcttcccacaggtggcatctgttttttggaaacacaatcatttcccatctcttcatgctcttccatatttctgtctgaatttctttgaaattcgtcttgggtaatatgtgatgtatgtatgttttcatctttagactgtcccacatcaagctgttcttcagctggtttagccatgaattttcttctctgtttttgttttatagtccttttgcttctagatggtttttctgcattcttggaatacatttcatattttgtagatctataattatttactgtttcacctatcaaagcataacttgtatccagtactgttttatcagagggctgagatgtctctactgggtgaggtttatgggaatgtttgtcatttgccaaagtcttaggtaatatattatgatgcttttctcttgactttctaccttgaaggagtgcagtgctctcagccggggatattgtgcgttgtttcagagaccctgcctttcttggtattgtaatccaagatctactggcaaaactttgatccgactcatcaattataaattcatcctctatcaacttcgtatcatcgggaggacacgaatgaggtggagcagttgccgcatgcctaacaatgggactggattcactttttcgttttactgtttctaaaaacaatgttgaaaaactttttttagcttgtcgttgaatttcatattctgaatctcgtattctattctgagatgatcctgatggttttctttcttgtccttccgatgttttatcctcttcatctgatactttattatctatttctattttctttaacataactttatcatcaaagtttaacctttttttggttttaactgaaacctctgtacttgaaggcagcatatttactgaattttcaaaagtgtaagtctctctcttttgggcactagatggaataacattttgtgatacagatgtttttgcatccaaaagaacagaaggtgagccaacggataagtaaaattcttcatcagcttcactgtgatgatcatttatgtttctacttgatatttttttcgagtcaggtgtatttttggaactaacatcagttgccagaattttctgatgaacttcatgggcctgaactgatctgtttgtggcttcacttggttctacaacaaactgtagagaggcttctttcttctttgaagaaactggaactgactttggatgtgatttctggcactctttgcttggtgactgaatacaagtgtcttttattttgcgtgttgaattaggcactgattttgtagaatttgtactaaaatcattggcaagacttttttcttcaaaacagtcttgtaagatttccagaacattctggccttgctctgtgttaatgtcacgtgccctggaaggtcgacaaaatcttcttctgtagccatttttgagatgatccagaccggacgcagccatgttccggccccgctgagccagcgcaactgtctgaggtggaagcccacacggaccacagctccaggaagccgagcaagaaacgaatcgccggaataccaggccgcggccaagcaataaccttaagtctcaggcgactgccgcgagagct

SEQ ID NO: 13786 - RNA, 5977 nt, Homo sapiens
  source 1..5977: mol_type = other RNA
gctgggattacaggcatgagccaccatgcccgggtagaagtctctttctttaagacccttcatgagcatgagggctgcctgacaaagtaggcaggactgtgattctttaaagacatgaaattaactccatagtcacccagttttatgcctgggggcactctccaaaactggacacagagagttaagctcaaaaagaacagtggtcttaatgggcacagaaagatcacaatttagggctgttgagaaaactgaattgtgatgcagggtacagaagtggaaactccactgaaaaagagctccagaaatctgcacgaggtgcccaagaacagaactttctgcaacttgtatctgtgacatctaatgtggtagccaccagtaccatgtgctactaagcacttgaaatgtggcaaatgcaagtaagaaacaatattttaaattaattttaaatagctacaacttgtgactactgtatcagccattatagccctagaagttggctgaacagttggctgaacagtaggctgcaaatgtgcagagcaaaattctgagacatgacagaagcctatgagctgaacagagtacagaggtggcaaaaatcagacgtggctctgaccaagcagaatggagagcctttgctgaaccatatgggctttcagtttagacaaagaaaggctacacttaagctgggcacagtggctcacacctgtaatcccaacactttgggaggctgaggtgggtggatcaccctgaggtcaggaattcgagacagccctggccaacatggtgaaaatctgtctctactaaaaacacaaaaactagccaggcgtggtggcaagcaactgtaatcccagctactcaggaggctgacgcaggagaattgcttgaacccgggaggtggaggttgcagtgagccgagatcacaccatcgcactccagcccaggcaacaagagtgaaactctgcctcaaaaaaaaaaaaaaagaaaagaaaagaaaaaagaaaataaagaaaaaatattgctaaagctttggaaaagaactgttggaatctgtggcctccttgagtgaggtctcacccacccctaggttgattggtaaaaactacagttttgtctggctgtagctaactgaaaaactagcaactttgccgtaagaggagtcttgatttacagcagaggtataaacctacaactttgtaagtcaaaagtaaaaaaatcacttaggaatggacaaggagtatctgtagttgctaaccaaaggttacagtcctagttcttgaagagcaacagagcagccagacatttaacaaggtcctggaaacagaagggcagaaaagggtaacatgagctctccaaacatctttggcaaactgaaatgatgcatgcacaggggagactcaagagagcatggcaaatgtaaaaaccaaggggaatttgggaactgcctcctacaatgaatgcatcccccatcccacacagaacaaccaacagtgggtggaaggcttatagactcaagtgtttgatcttaacctttgtccaaatgattggctgactgctaagctatgcagacacaggaactacccctagcaagcaagaataaatattgaaataaagaacttaaaaactgagcacagacagcaataacttcacatcatatataagatagattccacaatttgagtccagtcaaaatgctaaatttaaaacaatacaaatcccttagatataaaacaaaattgagttgctacaatatgctacctaaaatgtccagctgtcaaccaaaaattattagacatgtaaaaacatatgaaagtgaaatatactaaaggaaaaaaagcattcagtgaaaactaaatctgtatgggcccagatacttgattagtcaagccttcaataagacttcataacaaatatattcaaagaaataaaagtaaaaaaaaaattaaaaatgactcaataaaagagaaatcacaatagaaaattataaagtataaaaaaagagccatcacacttcattcttcctaagtcctacaccagagttgctttaaatgtgtgtatttaatggttaaataagacctgaaaagggagttggcctaaaaatatttttaccgtaaaacatcaatttcttcagagttaatgagaattatatgctaaccataccaaaaaccttgattagaatttttagcttagatgtattgattgatattaaaaagggaaagttgaggccacatacagaaagcaatggcgaaggacactgcctccaacagaaaatatgaaccaaaaagcataatggaaaaacatttacatgtaatatactaaatagatgtcatgccaacacagacacacaaggtgagaataccatgtgataatgcaagtagattgaaatgctaccggtgcaagccaaggaatgccagaaattgccagtaaaccaccagaagttaggaataaggaaggattctctcccttacaggttttcaaagacatcacggccttgacaacaccttgatttcagacttctagcctctagaactgagataataaatttctgttgctttaagtcactcattttgtggtattttgttacagcagttctaggaaattaatacaaacatgccttttaccacagttctctcccattggattatttaataataaatgatttaaaattagtatttggaaaagatgttttttaatgagtagacatattaatcaggtctcttttgacacagaaatgttctatatttcattttcatattcttgtcaaattataaaaataatatcataaatatggacatcgctacaagctattatgtacagtcactgaaaaatcagaaaaaacatgtgagttagaaatgtttatcaaatacaagtctacagaaaactgaataaaatttttattttaaaacatcacaagtaattacaaagacaaatattccaactatacaaactgtttttcacatatacatatatacatacatatatttaaggttggttgatctttcatctttttatctgagtaaaaagaagaacactttcctcattccggagatttttgatgttataatagttacctgaaggaacatagaacgaatccccagtacttaatatataaggtgtttcatgtaaagtacacaaaaggtcaccaaagttaacataaaaaaccaatatatcctggccaacatgctgctttcccttttcttcttgtggtcctaatatcaatttcccagtagaaaaaaagggtgtatccaatgtcttgtataccttcaactcaccatgcttaacaaaaaattgatatgtatcttgtggccttacaagatccatgagaataatctctcttgtttctgggtcctttaccctcgttggctgcaaaggatctccaagaggtatacctagatttaccattaagttagtctttctttcatcgttatcaagacagatccttttcttattagattttttgttgacttttccaatattttcttttgccttccttttagacgatattgtgtctggagatagtactccactaatcacgaatcctcctgatggccttccttgataatctattcgctctcctcgccagtactccaaaggtttcaaacgtgttctcttggtcctgcgaacatttggtgtgttggagggcaatactagtttgtgatggattctgttctttggtatcactttagattgttttgagtcatctgaacttccatgaacttcctcatcatccacatcattctttccagacattaaataattattattgagcctggaaggtccactttcctctaaaactgaagtcttatgctctccagaatccaagtttgactctgttggtatattacatgtatatccactggtctgaggctttaggggaacattctgtgcagtcataatgttatcttcattctttgagcttcttgtagatctagaacaatcaagatttttcttcttagccaagtctgcctcatcactttccaatggctcactcagcgaacatctggaaatttcatcatgaccaacgatacctccagaaccttcagcatttaaaaacttctgtactctttggttgcctttagttgctgtcttctgccttttaagtggaatagtttttttcctaatattcttagatgactgatttgttttcttagtagattttcggctactattgtgatgcattggtaattcatttcttactgaagaattgctataaacaggactctcctctgattttaccacccaccaatcagatggacgcctggaaattcttcgacttttcgtgacagttgaagtcacttcttcaggtacaagtttgttcttggactcactggaaaagcgcttctttttagattcttccttatcttttctagtgctacttttcttgcttcccacaggtggcatctgttttttggaaacacaatcatttcccatctcttcatgctcttccatatttctgtctgaatttctttgaaattcgtcttgggtaatatgtgatgtatgtatgttttcatctttagactgtcccacatcaagctgttcttcagctggtttagccatgaattttcttctctgtttttgttttatagtccttttgcttctagatggtttttctgcattcttggaatacatttcatattttgtagatctataattatttactgtttcacctatcaaagcataacttgtatccagtactgttttatcagagggctgagatgtctctactgggtgaggtttatgggaatgtttgtcatttgccaaagtcttaggtaatatattatgatgcttttctcttgactttctaccttgaaggagtgcagtgctctcagccggggatattgtgcgttgtttcagagaccctgcctttcttggtattgtaatccaagatctactggcaaaactttgatccgactcatcaattataaattcatcctctatcaacttcgtatcatcgggaggacacgaatgaggtggagcagttgccgcatgcctaacaatgggactggattcactttttcgttttactgtttctaaaaacaatgttgaaaaactttttttagcttgtcgttgaatttcatattctgaatctcgtattctattctgagatgatcctgatggttttctttcttgtccttccgatgttttatcctcttcatctgatactttattatctatttctattttctttaacataactttatcatcaaagtttaacctttttttggttttaactgaaacctctgtacttgaaggcagcatatttactgaattttcaaaagtgtaagtctctctcttttgggcactagatggaataacattttgtgatacagatgtttttgcatccaaaagaacagaaggtgagccaacggataagtaaaattcttcatcagcttcactgtgatgatcatttatgtttctacttgatatttttttcgagtcaggtgtatttttggaactaacatcagttgccagaattttctgatgaacttcatgggcctgaactgatctgtttgtggcttcacttggttctacaacaaactgtagagaggcttctttcttctttgaagaaactggaactgactttggatgtgatttctggcactctttgcttggtgactgaatacaagtgtcttttattttgcgtgttgaattaggcactgattttgtagaatttgtactaaaatcattggcaagacttttttcttcaaaacagtcttgtaagatttccagaacattctggccttgctctgtgttaatgtcacgtgccctggaaggtcgacaaaatcttcttctgtagccatttttgagatgatccagaccggacgcagccatgttccggccccgctgagccagcgcaactgtctgaggtggaagcccacacggaccacagctccaggaagccgagcaagaaacgaatcgccggaataccaggccgcggccaagcaataaccttaagtctcaggcgactgccgcgagagct

SEQ ID NO: 13787 - RNA, 5953 nt, Homo sapiens
  source 1..5953: mol_type = other RNA
gctgggattacaggcatgagccaccatgcccgggtagaagtctctttctttaagacccttcatgagcatgagggctgcctgacaaagtaggcaggactgtgattctttaaagacatgaaattaactccatagtcacccagttttatgcctgggggcactctccaaaactggacacagagagttaagctcaaaaagaacagtggtcttaatgggcacagaaagatcacaatttagggctgttgagaaaactgaattgtgatgcagggtacagaagtggaaactccactgaaaaagagctccagaaatctgcacgaggtgcccaagaacagaactttctgcaacttgtatctgtgacatctaatgtggtagccaccagtaccatgtgctactaagcacttgaaatgtggcaaatgcaagtaagaaacaatattttaaattaattttaaatagctacaacttgtgactactgtatcagccattatagccctagaagttggctgaacagttggctgaacagtaggctgcaaatgtgcagagcaaaattctgagacatgacagaagcctatgagctgaacagagtacagaggtggcaaaaatcagacgtggctctgaccaagcagaatggagagcctttgctgaaccatatgggctttcagtttagacaaagaaaggctacacttaagctgggcacagtggctcacacctgtaatcccaacactttgggaggctgaggtgggtggatcaccctgaggtcaggaattcgagacagccctggccaacatggtgaaaatctgtctctactaaaaacacaaaaactagccaggcgtggtggcaagcaactgtaatcccagctactcaggaggctgacgcaggagaattgcttgaacccgggaggtggaggttgcagtgagccgagatcacaccatcgcactccagcccaggcaacaagagtgaaactctgcctcaaaaaaaaaaaaaaagaaaagaaaagaaaaaagaaaataaagaaaaaatattgctaaagctttggaaaagaactgttggaatctgtggcctccttgagtgaggtctcacccacccctaggttgattggtaaaaactacagttttgtctggctgtagctaactgaaaaactagcaactttgccgtaagaggagtcttgatttacagcagaggtataaacctacaactttgtaagtcaaaagtaaaaaaatcacttaggaatggacaaggagtatctgtagttgctaaccaaaggttacagtcctagttcttgaagagcaacagagcagccagacatttaacaaggtcctggaaacagaagggcagaaaagggtaacatgagctctccaaacatctttggcaaactgaaatgatgcatgcacaggggagactcaagagagcatggcaaatgtaaaaaccaaggggaatttgggaactgcctcctacaatgaatgcatcccccatcccacacagaacaaccaacagtgggtggaaggcttatagactcaagtgtttgatcttaacctttgtccaaatgattggctgactgctaagctatgcagacacaggaactacccctagcaagcaagaataaatattgaaataaagaacttaaaaactgagcacagacagcaataacttcacatcatatataagatagattccacaatttgagtccagtcaaaatgctaaatttaaaacaatacaaatcccttagatataaaacaaaattgagttgctacaatatgctacctaaaatgtccagctgtcaaccaaaaattattagacatgtaaaaacatatgaaagtgaaatatactaaaggaaaaaaagcattcagtgaaaactaaatctgtatgggcccagatacttgattagtcaagccttcaataagacttcataacaaatatattcaaagaaataaaagtaaaaaaaaaattaaaaatgactcaataaaagagaaatcacaatagaaaattataaagtataaaaaaagagccatcacacttcattcttcctaagtcctacaccagagttgctttaaatgtgtgtatttaatggttaaataagacctgaaaagggagttggcctaaaaatatttttaccgtaaaacatcaatttcttcagagttaatgagaattatatgctaaccataccaaaaaccttgattagaatttttagcttagatgtattgattgatattaaaaagggaaagttgaggccacatacagaaagcaatggcgaaggacactgcctccaacagaaaatatgaaccaaaaagcataatggaaaaacatttacatgtaatatactaaatagatgtcatgccaacacagacacacaaggtgagaataccatgtgataatgcaagtagattgaaatgctaccggtgcaagccaaggaatgccagaaattgccagtaaaccaccagaagttaggaataaggaaggattctctcccttacaggttttcaaagacatcacggccttgacaacaccttgatttcagacttctagcctctagaactgagataataaatttctgttgctttaagtcactcattttgtggtattttgttacagcagttctaggaaattaatacaaacatgccttttaccacagttctctcccattggattatttaataataaatgatttaaaattagtatttggaaaagatgttttttaatgagtagacatattaatcaggtctcttttgacacagaaatgttctatatttcattttcatattcttgtcaaattataaaaataatatcataaatatggacatcgctacaagctattatgtacagtcactgaaaaatcagaaaaaacatgtgagttagaaatgtttatcaaatacaagtctacagaaaactgaataaaatttttattttaaaacatcacaagtaattacaaagacaaatattccaactatacaaactgtttttcacatatacatatatacatacatatatttaaggttggttgatctttcatctttttatctgagtaaaaagaagaacactttcctcattccggagatttttgatgttataatagttacctgaaggaacatagaacgaatccccagtacttaatatataaggtgtttcatgtaaagtacacaaaaggtcaccaaagttaacataaaaaaccaatatatcctggccaacatgctgctttcccttttcttcttgtggtcctaatatcaatttcccagtagaaaaaaagggtgtatccaatgtcttgtataccttcaactcaccatgcttaacaaaaaattgatatgtatcttgtggccttacaagatccatgagaataatctctcttgtttctgggtcctttaccctcgttggctgcaaaggatctccaagaggtatacttctttcatcgttatcaagacagatccttttcttattagattttttgttgacttttccaatattttcttttgccttccttttagacgatattgtgtctggagatagtactccactaatcacgaatcctcctgatggccttccttgataatctattcgctctcctcgccagtactccaaaggtttcaaacgtgttctcttggtcctgcgaacatttggtgtgttggagggcaatactagtttgtgatggattctgttctttggtatcactttagattgttttgagtcatctgaacttccatgaacttcctcatcatccacatcattctttccagacattaaataattattattgagcctggaaggtccactttcctctaaaactgaagtcttatgctctccagaatccaagtttgactctgttggtatattacatgtatatccactggtctgaggctttaggggaacattctgtgcagtcataatgttatcttcattctttgagcttcttgtagatctagaacaatcaagatttttcttcttagccaagtctgcctcatcactttccaatggctcactcagcgaacatctggaaatttcatcatgaccaacgatacctccagaaccttcagcatttaaaaacttctgtactctttggttgcctttagttgctgtcttctgccttttaagtggaatagtttttttcctaatattcttagatgactgatttgttttcttagtagattttcggctactattgtgatgcattggtaattcatttcttactgaagaattgctataaacaggactctcctctgattttaccacccaccaatcagatggacgcctggaaattcttcgacttttcgtgacagttgaagtcacttcttcaggtacaagtttgttcttggactcactggaaaagcgcttctttttagattcttccttatcttttctagtgctacttttcttgcttcccacaggtggcatctgttttttggaaacacaatcatttcccatctcttcatgctcttccatatttctgtctgaatttctttgaaattcgtcttgggtaatatgtgatgtatgtatgttttcatctttagactgtcccacatcaagctgttcttcagctggtttagccatgaattttcttctctgtttttgttttatagtccttttgcttctagatggtttttctgcattcttggaatacatttcatattttgtagatctataattatttactgtttcacctatcaaagcataacttgtatccagtactgttttatcagagggctgagatgtctctactgggtgaggtttatgggaatgtttgtcatttgccaaagtcttaggtaatatattatgatgcttttctcttgactttctaccttgaaggagtgcagtgctctcagccggggatattgtgcgttgtttcagagaccctgcctttcttggtattgtaatccaagatctactggcaaaactttgatccgactcatcaattataaattcatcctctatcaacttcgtatcatcgggaggacacgaatgaggtggagcagttgccgcatgcctaacaatgggactggattcactttttcgttttactgtttctaaaaacaatgttgaaaaactttttttagcttgtcgttgaatttcatattctgaatctcgtattctattctgagatgatcctgatggttttctttcttgtccttccgatgttttatcctcttcatctgatactttattatctatttctattttctttaacataactttatcatcaaagtttaacctttttttggttttaactgaaacctctgtacttgaaggcagcatatttactgaattttcaaaagtgtaagtctctctcttttgggcactagatggaataacattttgtgatacagatgtttttgcatccaaaagaacagaaggtgagccaacggataagtaaaattcttcatcagcttcactgtgatgatcatttatgtttctacttgatatttttttcgagtcaggtgtatttttggaactaacatcagttgccagaattttctgatgaacttcatgggcctgaactgatctgtttgtggcttcacttggttctacaacaaactgtagagaggcttctttcttctttgaagaaactggaactgactttggatgtgatttctggcactctttgcttggtgactgaatacaagtgtcttttattttgcgtgttgaattaggcactgattttgtagaatttgtactaaaatcattggcaagacttttttcttcaaaacagtcttgtaagatttccagaacattctggccttgctctgtgttaatgtcacgtgccctggaaggtcgacaaaatcttcttctgtagccatttttgagatgatccagaccggacgcagccatgttccggccccgctgagccagcgcaactgtctgaggtggaagcccacacggaccacagctccaggaagccgagcaagaaacgaatcgccggaataccaggccgcggccaagcaataaccttaagtctcaggcgactgccgcgagagct

SEQ ID NO: 13788 - RNA, 5803 nt, Homo sapiens
  source 1..5803: mol_type = other RNA
gctgggattacaggcatgagccaccatgcccggtctacttccttcctttctaagaagtctttcttcatgtcaaagccaacttctgcccaggatctgaatatttagaaatgcattgtccaatataatagccactagccacaggtagccaaatttaaatgaactacaatgaaatacaattaaattttagcccctcagccacactagccatgttttgagtgcttgactgccacatgtggctaatgtactagacatcattaccaaaagttctgttggaaagccctgctctaaagtaaattatattgcctatataatcttcctaccaatacactcttttgcccctgaaaatgactcctcctcttcacttcttaacactcaaaatgtaccctcaaattactaaagtatcaatgcatgtcccattttcagttatcttccttcttagcctctctgttgaaaaaccactagaaagcatccaacccggaactttttaaagaactactcaaccgtcttctttccctccaatcagttccatttggttcctcctcttacataacgttttcctcattgtttaatttttttttgagacagagtcttgctctgtcacccaggctggaatgccgtggcacaatctcagctcactacaagctccgcctcccgggttcacgccattctcctgcctcagcctcccaagtagttgggactacaggtgcccgcaaccacgcccagctaattttttgtatttttagtagagacggggtttcaacgtgtcagccaggatggtcttgatctcctgacctcgtgatccgcccacctcggcctcccaaagtgctgggattacaggcgtgagccaccgtgcctggcctcttttttttgtatttgcaattgtccttcatggttctaatttacctccatggcataaactacctgtaccccatatggattcccaactctcttatgtcaacctctctgcctcacgccctagaattttgttttcacccagatacctgccagattgtcagccgtatcttctttcccttcccccagctccccaaaccaggacaacatgatctccctacatctttaaccccaccactttcctactctttttttggggggggtctcattctgccacccaggatggagtgcagcagtgtgatcacagcttgctgcagcctcagactcctgggctcaaaggatcctctggcttcggccctccaagtagataggactgcaggcacgcaccaccatgtttggctaagtttttatattttgtagagacaggttctcactttattgccaggctggtctcgaactcctggattcaagaaatcctctcacctcagcctcctaaagtgcagggattacaggcatgagccactgcacccggctaattctcctactctaaaaaccagtcatccttgtctttcctcctcacatcaagtggccaggcctttcacaatgcctgtctttatttagtgctatctctcctgccactactctagctcagaccctgattattctctcctagaaaactaaattaacctaacccaattttttccaaagtgtggtgtattcactgctatagttactttaatgtgattaggaaaaaacactaacacatcaaaactttgatttcaaaatagaattgtgtcaagtaagaacaaaataaatctggaaatgagtagatctgaagaaaacaatgtaggcagcaatgaatatggaaaaagccatcaaaaatggtaacataaatggctgaaatgtgagaaacaccatgttagtgaatcactttgctaatctgcaaattagttaccaaattaattcttcttatatgttattcagatcacaacatatcctattcaaaatctccagtggcatccccattaactccaagtaaaattataactcctcagcctcattttaagacacaacctgttccctactctgtctaaatctacctttagagctattgtggccttctcatctctatcaatgcctttattattttgtttctctttaaatggaatgctcaggccaggtgcagtggctcacgcctgtaatcccaacactttgggaggcagaggcgggtggatcacttgaggtcaggagttcgcgaccagcctggccaacatgctgaaaccccgtccgtactaaaaatacaaaaatcagctgggcatggtggtgggtatctgtaatcacagctcctcgggaagctgagacaggagaatcgcttgaactcaagaagcagaggttgcagtgagccatgatctcaccactgcactccatccagcctgggtgacagagcgagactccatctcaaaaagagaaaaataaataaataatggaatgctcaatattcactatcccacaacccaactctgcttgtcaaaaatccacttttggaacccaataaaaatgaatatgcaagtttaacatgttggctgggcgcagtggctcaagcctgtaatcccatcactttgggaggctgaggtgggtggatcacttgaggtcaggagttccagaccagcctggccaacatggtgaaacctcacctctactaataatacaaaaattagctgggtgtggtggcaggcgcctgtgatctcagctactcgggaggctgaggtgggagaactgcttgaacccaggaggcagaggttgcagtgagctgagatcaggccactgaactccagcctaggtgacaagagtcaaactccgtctcaaaaaaaaaaaaaaaaagaaaaaaagaaaaaagttttaacatgtttatgaagtacccattacatgccttcttccatgagtttttccaattcattcccactaggatcaatctcgtcccctctactcaattcccataacactattatttgtggcattcatcacacagtatctgtagctttatgtatgttttctctcctagtagattctaagcaacttgagagtaggaatggtgcctccatctttatttctgtctccatcttaatatcctatacctagaagataccaggaagtgtcagctgaataaatgaatctgaaccttaatctcaaaggctatgcggcagtaagaaatggaatggacaaaaggaaacgtgaatttgatatgacttaaagttttagattaaggaaaacttccctacctgattatatctgtttaaaagaagagcaaaagtgtttttaacagatggaatcttgctgtgttgcccaggctggagtactacagtggctatttataggtgcaatcccactactgatcagcacaggaattttgacctgctccatttccgacctgggccagttcaccccttcttaggcaaccttgttgttctccactcccaggaggtcaccatactgatgccaaatttagtgaggacatctgacctgcatagcacactacagtgcagaactcctgggctcaagcaatcctcctgcctcagcctcccaagaagctacaggcagtacaggcaagtgccattgcacccagctaaaagaaaagcaaattttaaatacataccctgctgggaaactaaagtactaagtgaacaacacttacgtgcttggattagtataattcacagctatactattaagaaatctctgctgtgtaaattggaatgcgaattccttttttttttttgagatggagtctctctgttgcccaggctggaatgcagtggcgcgatctccgctcactgcaacctccgcctcccaggtgcaagcgattctcctgcctcagcctcccgagtagctgggattacaggcacccacccaccatgcccagctaatttttgtatttttagtagagacggggtttcaccatgttggccgagctggtctcgaactcatgacctcaggtgatccacctgccccagcctcccaaagtgctgggattataggcgtgagctaccacgcccggcctataatgggaatttctaaaatgttgatatttaattccacaatatgaaccaaggaaaattttactagcagaaatttatgtatgtaataaatcattagcctcatatgcacattatttgaaatatgcatgattggtcattttagttttcccaataataatttatcacttatcttatatcccactagtcacacactagcaggcaaatggtagcaagtctcaaatatgtaagaaaggtttaaagaagaaaaagtaaaaaaaccgtccagaattctatccattgtgtatttttctgtgactggagttgacataattagtcaatcttagcaataatgtattgggttcactgggtgttctgaggatgcaccatttgaaccaccggtaaaagggtacagaatgtgtattgagagtcacttcaatggcttctcaatgacaccacaccaaaggaggaatacctgaagagagaatggaaacactgcaggcaggatgatttaagaacctggaaataaggaatttaatcttgttcagcttgaggagtataactaaaattactatcctgagtaacctgtactaaatccatcactctggtagaatcagatcagctgagtttaaatgtcaagaaaaaatagacacacacaaaagtggctttgattacataagtcagaggagggggagcctacaatagctcttccccacatcacacccccaaggctccttcttagggacagcaacagctttgtcaatgacacaaatgcagggtggcatgaggtttccagcagcttaacattttaatttggggtgggggtggaagaaaatacataagttgctttttgctcccccatcctaatgccttggggaccagccaggctgacccaaatggaatccagagcgagagtggggccttgggttccccgaggagtaaagggggcagatccagaacagagcagaaacggtgataattatatagaggtcatgtcattgagggcgtggtccagctcctcgctaatggccttgtacttcagtttctgggcatagagctcatcttccaggtcatcaattgtcttttccagcttggctaccgatctctcagcaaactcagcacgggtctctgcctccttgagtttatcagtaagaatcttgatttcttcctcatatttatcttctttttgagagtacttctccgcctgagcctcaagagacttgaggttgttggtgacattcttcagctcctcctccagctcagaacacttagactctgccagctcagctcgttcctctgtgcgttccaagtctccttcaatgatcaccaacttacgagccacctcttcatacttcctatctgcctcttctgcaatgtgcttagcttctttgagttggatttcctggagttccatcttttcttcatcttttaaggcccggttttcaataaccttcatacctctctcactctcatcagcagctttttcagcttcttccagcttttgcagggcagtggccaggcgctcctgagcacggtccagctcttcttcaaccagctggatcctacggttcaaggaggccacctcagcctcagcatcagcagccttcttctctgccagttccagcttctcctgggcatccttcaaagcttcagaatacttgtccagctcatcctctgtccctttcagcttcttctgcatggctgccagctcatcctccagctgtttacttctttcttctgcctgcttctgctcagcttcagcttgctctgcccgatccagagcattctccttgtctaacttcagcatctgcatctttttcttgatggcctccatcatgagcagtggctgttggtaggctcacctgtgaacactggagaactggagactggggcaagaaagaaggggctgctgcctgagt

SEQ ID NO: 13789 - RNA, 5803 nt, Homo sapiens
  source 1..5803: mol_type = other RNA
gctgggattacaggcatgagccaccatgcccggtctacttccttcctttctaagaagtctttcttcatgtcaaagccaacttctgcccaggatctgaatatttagaaatgcattgtccaatataatagccactagccacaggtagccaaatttaaatgaactacaatgaaatacaattaaattttagcccctcagccacactagccatgttttgagtgcttgactgccacatgtggctaatgtactagacatcattaccaaaagttctgttggaaagccctgctctaaagtaaattatattgcctatataatcttcctaccaatacactcttttgcccctgaaaatgactcctcctcttcacttcttaacactcaaaatgtaccctcaaattactaaagtatcaatgcatgtcccattttcagttatcttccttcttagcctctctgttgaaaaaccactagaaagcatccaacccggaactttttaaagaactactcaaccgtcttctttccctccaatcagttccatttggttcctcctcttacataacgttttcctcattgtttaatttttttttgagacagagtcttgctctgtcacccaggctggaatgccgtggcacaatctcagctcactacaagctccgcctcccgggttcacgccattctcctgcctcagcctcccaagtagttgggactacaggtgcccgcaaccacgcccagctaattttttgtatttttagtagagacggggtttcaacgtgtcagccaggatggtcttgatctcctgacctcgtgatccgcccacctcggcctcccaaagtgctgggattacaggcgtgagccaccgtgcctggcctcttttttttgtatttgcaattgtccttcatggttctaatttacctccatggcataaactacctgtaccccatatggattcccaactctcttatgtcaacctctctgcctcacgccctagaattttgttttcacccagatacctgccagattgtcagccgtatcttctttcccttcccccagctccccaaaccaggacaacatgatctccctacatctttaaccccaccactttcctactctttttttggggggggtctcattctgccacccaggatggagtgcagcagtgtgatcacagcttgctgcagcctcagactcctgggctcaaaggatcctctggcttcggccctccaagtagataggactgcaggcacgcaccaccatgtttggctaagtttttatattttgtagagacaggttctcactttattgccaggctggtctcgaactcctggattcaagaaatcctctcacctcagcctcctaaagtgcagggattacaggcatgagccactgcacccggctaattctcctactctaaaaaccagtcatccttgtctttcctcctcacatcaagtggccaggcctttcacaatgcctgtctttatttagtgctatctctcctgccactactctagctcagaccctgattattctctcctagaaaactaaattaacctaacccaattttttccaaagtgtggtgtattcactgctatagttactttaatgtgattaggaaaaaacactaacacatcaaaactttgatttcaaaatagaattgtgtcaagtaagaacaaaataaatctggaaatgagtagatctgaagaaaacaatgtaggcagcaatgaatatggaaaaagccatcaaaaatggtaacataaatggctgaaatgtgagaaacaccatgttagtgaatcactttgctaatctgcaaattagttaccaaattaattcttcttatatgttattcagatcacaacatatcctattcaaaatctccagtggcatccccattaactccaagtaaaattataactcctcagcctcattttaagacacaacctgttccctactctgtctaaatctacctttagagctattgtggccttctcatctctatcaatgcctttattattttgtttctctttaaatggaatgctcaggccaggtgcagtggctcacgcctgtaatcccaacactttgggaggcagaggcgggtggatcacttgaggtcaggagttcgcgaccagcctggccaacatgctgaaaccccgtccgtactaaaaatacaaaaatcagctgggcatggtggtgggtatctgtaatcacagctcctcgggaagctgagacaggagaatcgcttgaactcaagaagcagaggttgcagtgagccatgatctcaccactgcactccatccagcctgggtgacagagcgagactccatctcaaaaagagaaaaataaataaataatggaatgctcaatattcactatcccacaacccaactctgcttgtcaaaaatccacttttggaacccaataaaaatgaatatgcaagtttaacatgttggctgggcgcagtggctcaagcctgtaatcccatcactttgggaggctgaggtgggtggatcacttgaggtcaggagttccagaccagcctggccaacatggtgaaacctcacctctactaataatacaaaaattagctgggtgtggtggcaggcgcctgtgatctcagctactcgggaggctgaggtgggagaactgcttgaacccaggaggcagaggttgcagtgagctgagatcaggccactgaactccagcctaggtgacaagagtcaaactccgtctcaaaaaaaaaaaaaaaaagaaaaaaagaaaaaagttttaacatgtttatgaagtacccattacatgccttcttccatgagtttttccaattcattcccactaggatcaatctcgtcccctctactcaattcccataacactattatttgtggcattcatcacacagtatctgtagctttatgtatgttttctctcctagtagattctaagcaacttgagagtaggaatggtgcctccatctttatttctgtctccatcttaatatcctatacctagaagataccaggaagtgtcagctgaataaatgaatctgaaccttaatctcaaaggctatgcggcagtaagaaatggaatggacaaaaggaaacgtgaatttgatatgacttaaagttttagattaaggaaaacttccctacctgattatatctgtttaaaagaagagcaaaagtgtttttaacagatggaatcttgctgtgttgcccaggctggagtactacagtggctatttataggtgcaatcccactactgatcagcacaggaattttgacctgctccatttccgacctgggccagttcaccccttcttaggcaaccttgttgttctccactcccaggaggtcaccatactgatgccaaatttagtgaggacatctgacctgcatagcacactacagtgcagaactcctgggctcaagcaatcctcctgcctcagcctcccaagaagctacaggcagtacaggcaagtgccattgcacccagctaaaagaaaagcaaattttaaatacataccctgctgggaaactaaagtactaagtgaacaacacttacgtgcttggattagtataattcacagctatactattaagaaatctctgctgtgtaaattggaatgcgaattccttttttttttttgagatggagtctctctgttgcccaggctggaatgcagtggcgcgatctccgctcactgcaacctccgcctcccaggtgcaagcgattctcctgcctcagcctcccgagtagctgggattacaggcacccacccaccatgcccagctaatttttgtatttttagtagagacggggtttcaccatgttggccgagctggtctcgaactcatgacctcaggtgatccacctgccccagcctcccaaagtgctgggattataggcgtgagctaccacgcccggcctataatgggaatttctaaaatgttgatatttaattccacaatatgaaccaaggaaaattttactagcagaaatttatgtatgtaataaatcattagcctcatatgcacattatttgaaatatgcatgattggtcattttagttttcccaataataatttatcacttatcttatatcccactagtcacacactagcaggcaaatggtagcaagtctcaaatatgtaagaaaggtttaaagaagaaaaagtaaaaaaaccgtccagaattctatccattgtgtatttttctgtgactggagttgacataattagtcaatcttagcaataatgtattgggttcactgggtgttctgaggatgcaccatttgaaccaccggtaaaagggtacagaatgtgtattgagagtcacttcaatggcttctcaatgacaccacaccaaaggaggaatacctgaagagagaatggaaacactgcaggcaggatgatttaagaacctggaaataaggaatttaatcttgttcagcttgaggagtataactaaaattactatcctgagtaacctgtactaaatccatcactctggtagaatcagatcagctgagtttaaatgtcaagaaaaaatagacacacacaaaagtggctttgattacataagtcagaggagggggagcctacaatagctcttccccacatcacacccccaaggctccttcttagggacagcaacagctttgtcaatgacacaaatgcagggtggcatgaggtttccagcagcttaacattttaatttggggtgggggtggaagaaaatacataagttgctttttgctcccccatcctaatgccttggggaccagccaggctgacccaaatggaatccagagcgagagtggggccttgggttccccgaggagtaaagggggcagatccagaacagagcagaaacggtgataattatatagaggtcatgtcattgagggcgtggtccagctcctcgctaatggccttgtacttcagtttctgggcatagagctcatcttccaggtcatcaattgtcttttccagcttggctaccgatctctcagcaaactcagcacgggtctctgcctccttgagtttatcagtaagaatcttgatttcttcctcatatttatcttctttttgagagtacttttcttcagcagcactcagacacttcaggttctggtccatcagtctaatctgctcatccatctctcggcaacgggactctgccagctcagctcgttcctctgtgcgttccaagtctccttcaatgatcaccaacttacgagccacctcttcatacttcctatctgcctcttctgcaatgtgcttagcttctttgagttggatttcctggagttccatcttttcttcatcttttaaggcccggttttcaataaccttcatacctctctcactctcatcagcagctttttcagcttcttccagcttttgcagggcagtggccaggcgctcctgagcacggtccagctcttcttcaaccagctggatcctacggttcaaggaggccacctcagcctcagcatcagcagccttcttctctgccagttccagcttctcctgggcatccttcaaagcttcagaatacttgtccagctcatcctctgtccctttcagcttcttctgcatggctgccagctcatcctccagctgtttacttctttcttctgcctgcttctgctcagcttcagcttgctctgcccgatccagagcattctccttgtctaacttcagcatctgcatctttttcttgatggcctccatcatgagcagtggctgttggtaggctcacctgtgaacactggagaactggagactggggcaagaaagaaggggctgctgcctgagt

SEQ ID NO: 13790 - RNA, 5709 nt, Homo sapiens
  source 1..5709: mol_type = other RNA
gctgggattacaggcatgagccaccatgcccggtctacttccttcctttctaagaagtctttcttcatgtcaaagccaacttctgcccaggatctgaatatttagaaatgcattgtccaatataatagccactagccacaggtagccaaatttaaatgaactacaatgaaatacaattaaattttagcccctcagccacactagccatgttttgagtgcttgactgccacatgtggctaatgtactagacatcattaccaaaagttctgttggaaagccctgctctaaagtaaattatattgcctatataatcttcctaccaatacactcttttgcccctgaaaatgactcctcctcttcacttcttaacactcaaaatgtaccctcaaattactaaagtatcaatgcatgtcccattttcagttatcttccttcttagcctctctgttgaaaaaccactagaaagcatccaacccggaactttttaaagaactactcaaccgtcttctttccctccaatcagttccatttggttcctcctcttacataacgttttcctcattgtttaatttttttttgagacagagtcttgctctgtcacccaggctggaatgccgtggcacaatctcagctcactacaagctccgcctcccgggttcacgccattctcctgcctcagcctcccaagtagttgggactacaggtgcccgcaaccacgcccagctaattttttgtatttttagtagagacggggtttcaacgtgtcagccaggatggtcttgatctcctgacctcgtgatccgcccacctcggcctcccaaagtgctgggattacaggcgtgagccaccgtgcctggcctcttttttttgtatttgcaattgtccttcatggttctaatttacctccatggcataaactacctgtaccccatatggattcccaactctcttatgtcaacctctctgcctcacgccctagaattttgttttcacccagatacctgccagattgtcagccgtatcttctttcccttcccccagctccccaaaccaggacaacatgatctccctacatctttaaccccaccactttcctactctttttttggggggggtctcattctgccacccaggatggagtgcagcagtgtgatcacagcttgctgcagcctcagactcctgggctcaaaggatcctctggcttcggccctccaagtagataggactgcaggcacgcaccaccatgtttggctaagtttttatattttgtagagacaggttctcactttattgccaggctggtctcgaactcctggattcaagaaatcctctcacctcagcctcctaaagtgcagggattacaggcatgagccactgcacccggctaattctcctactctaaaaaccagtcatccttgtctttcctcctcacatcaagtggccaggcctttcacaatgcctgtctttatttagtgctatctctcctgccactactctagctcagaccctgattattctctcctagaaaactaaattaacctaacccaattttttccaaagtgtggtgtattcactgctatagttactttaatgtgattaggaaaaaacactaacacatcaaaactttgatttcaaaatagaattgtgtcaagtaagaacaaaataaatctggaaatgagtagatctgaagaaaacaatgtaggcagcaatgaatatggaaaaagccatcaaaaatggtaacataaatggctgaaatgtgagaaacaccatgttagtgaatcactttgctaatctgcaaattagttaccaaattaattcttcttatatgttattcagatcacaacatatcctattcaaaatctccagtggcatccccattaactccaagtaaaattataactcctcagcctcattttaagacacaacctgttccctactctgtctaaatctacctttagagctattgtggccttctcatctctatcaatgcctttattattttgtttctctttaaatggaatgctcaggccaggtgcagtggctcacgcctgtaatcccaacactttgggaggcagaggcgggtggatcacttgaggtcaggagttcgcgaccagcctggccaacatgctgaaaccccgtccgtactaaaaatacaaaaatcagctgggcatggtggtgggtatctgtaatcacagctcctcgggaagctgagacaggagaatcgcttgaactcaagaagcagaggttgcagtgagccatgatctcaccactgcactccatccagcctgggtgacagagcgagactccatctcaaaaagagaaaaataaataaataatggaatgctcaatattcactatcccacaacccaactctgcttgtcaaaaatccacttttggaacccaataaaaatgaatatgcaagtttaacatgttggctgggcgcagtggctcaagcctgtaatcccatcactttgggaggctgaggtgggtggatcacttgaggtcaggagttccagaccagcctggccaacatggtgaaacctcacctctactaataatacaaaaattagctgggtgtggtggcaggcgcctgtgatctcagctactcgggaggctgaggtgggagaactgcttgaacccaggaggcagaggttgcagtgagctgagatcaggccactgaactccagcctaggtgacaagagtcaaactccgtctcaaaaaaaaaaaaaaaaagaaaaaaagaaaaaagttttaacatgtttatgaagtacccattacatgccttcttccatgagtttttccaattcattcccactaggatcaatctcgtcccctctactcaattcccataacactattatttgtggcattcatcacacagtatctgtagctttatgtatgttttctctcctagtagattctaagcaacttgagagtaggaatggtgcctccatctttatttctgtctccatcttaatatcctatacctagaagataccaggaagtgtcagctgaataaatgaatctgaaccttaatctcaaaggctatgcggcagtaagaaatggaatggacaaaaggaaacgtgaatttgatatgacttaaagttttagattaaggaaaacttccctacctgattatatctgtttaaaagaagagcaaaagtgtttttaacagatggaatcttgctgtgttgcccaggctggagtactacagtggctatttataggtgcaatcccactactgatcagcacaggaattttgacctgctccatttccgacctgggccagttcaccccttcttaggcaaccttgttgttctccactcccaggaggtcaccatactgatgccaaatttagtgaggacatctgacctgcatagcacactacagtgcagaactcctgggctcaagcaatcctcctgcctcagcctcccaagaagctacaggcagtacaggcaagtgccattgcacccagctaaaagaaaagcaaattttaaatacataccctgctgggaaactaaagtactaagtgaacaacacttacgtgcttggattagtataattcacagctatactattaagaaatctctgctgtgtaaattggaatgcgaattccttttttttttttgagatggagtctctctgttgcccaggctggaatgcagtggcgcgatctccgctcactgcaacctccgcctcccaggtgcaagcgattctcctgcctcagcctcccgagtagctgggattacaggcacccacccaccatgcccagctaatttttgtatttttagtagagacggggtttcaccatgttggccgagctggtctcgaactcatgacctcaggtgatccacctgccccagcctcccaaagtgctgggattataggcgtgagctaccacgcccggcctataatgggaatttctaaaatgttgatatttaattccacaatatgaaccaaggaaaattttactagcagaaatttatgtatgtaataaatcattagcctcatatgcacattatttgaaatatgcatgattggtcattttagttttcccaataataatttatcacttatcttatatcccactagtcacacactagcaggcaaatggtagcaagtctcaaatatgtaagaaaggtttaaagaagaaaaagtaaaaaaaccgtccagaattctatccattgtgtatttttctgtgactggagttgacataattagtcaatcttagcaataatgtattgggttcactgggtgttctgaggatgcaccatttgaaccaccggtaaaagggtacagaatgtgtattgagagtcacttcaatggcttctcaatgacaccacaccaaaggaggaatacctgaagagagaatggaaacactgcaggcaggatgatttaagaacctggaaataaggaatttaatcttgttcagcttgaggagtataactaaaattactatcctgagtaacctgtactaaatccatcactctggtagaatcagatcagctgagtttaaatgtcaagaaaaaatagacacacacaaaagtggctttgattacataagtcagaggagggggagcctacaatagctcttccccacatcacacccccaaggctccttcttagggacagcaacagctttgtcaatgacacaaatgcagggtggcatgaggtttccagcagcttaacattttaatttggggtgggggtggaagaaaatacataagttgctttttgctcccccatcctaatgccttggggaccagccaggctgacccaaatggaatccagagcgagagtggggccttgggttccccgaggagtaaagggggcagatccagaacagagcagaaacggtgataattatatagaggtcatgtcattgagggcgtggtccagctcctcgctaatggccttgtacttcagtttctgggcatagagctcatcttccaggtcatcaattgtcttttccagcttggctaccgatctctcagcaaactcagcacgggtctctgcctccttgagtttatcagtaagaatcttgatttcttcctcatatttatcttctttttgagagtacttttcttcagcagcactcagacacttcaggttctggtccatcagtctaatctgctcatccatctctcggcaacgggactctgccagctcagctcgttcctctgtgcgttccaagtctccttcaatgatcaccaacttacgagccacctcttcatacttcctatctgcctcttctgcaatgtgcttagcttctttgagttggatttcctggagttccatcttttcttcatcttttaaggcccggttttcaataaccttcatacctctctcactctcatcagcagctttttcagcttcttccagcttttgcagggcagtggccaggcgctcctgagcacggtccagctcttcttcaaccagctggatcctacggttcaaggaggccacctcagcctcagcctgttcccgggcccgcctttctccctcaacttctcgctggaggcgctcagctcgctcctctgcatcatctgcctgctgctgcagaacctggatcttgcgcttcaccgcctcgatggtggtgatcccagccatggtgcccacccagctactgctcgcgctccggttcctgcctcctccgctcggcgttgcagcctcctctcacccttacttccgcctgctacgccctgaaat

SEQ ID NO: 13791 - RNA, 1294 nt, Homo sapiens
  source 1..1294: mol_type = other RNA
gctgggattacaggcatgagccaccatgcccgtcctcaattctttaactttgcctcagtccaaagagagcatttataaagtcaagtgtgtgaaaaccatagttgtctaatgcggagttttaaaagacctgtctttttgagagaaacaatgtgcgttcacatttaggttccggaagatctcaaagagttccagaccacagatattccggtgcatcactgtaacttccgggctgttctcggctgcctttgtagcgcttctgttctcggtagctacgcagggccagcaccacgctggcgccgtacatgatcacgagaagacaagcaaaggtggctgctgctccgtcggtgcctgccagctggcagtccatccaggtgagacccttgcgggcatagagcctctctcttgttttgcaagtgtcggtgctattgatctgcagagccacgtggaggtaaacaccaatgcctgtgcagtagcccactgccgctaggaggctgaaggcggcctccgtgaggagccacttccctgacaacattgttcgactcttggctccttggagtaaaacacccatggtgaggacccccagacccagagaaacagccacgccaccgtatatcaggggcgagcggaggatcgtgtactgctggtccagctgccgaacctgctctagctcagtgccctcgaacggtgagtagtagttgttcccaaagccaccgccgctggaaaagctggcactgaatccggcaaggacaaagtaggaggccacgatgcatatgagaaccatcccattcaagaccacctccactatctgcaccacacctctcccagtgcacaagtatttgcatttgtggcattccaggagtccttccgcctctgactggtaatattccacctcctctcgtccaggcctgggggtcgagggcagatatctctccgaagggggttcactgcgcgagggcccgcgtccctgtgtgtgtcccggcgggggcctcggtccgggtctctttccctctctctctccctctcccggtcccggttccggtcgcggttcccgtccctctcctggtctctctccgggtcccggtccccgtcccttcgccggttcccgtcgctgcttcgcttcctgcgcgggtccccgggtcggtcccgcggtcgatcgtgggtgcggccttggtctgggtgggggcgccgtcccgggtcccgctctctcggccgggcccggggctcgcgagcccccgacggatcttccatggccgggttccgtgtccccgcccgggagcgacctgagggcaacaac

SEQ ID NO: 13792 - RNA, 1457 nt, Homo sapiens
  source 1..1457: mol_type = other RNA
gctgggattacaggcatgagccaccatgcccgtcctcaattctttaactttgcctcagtccaaagagagcatttataaagtcaagtgtgtgaaaaccatagttgtctaatgcggagttttaaaagacctgtctttttgagagaaacaatgtgcgttcacatttaggttccggaagatctcaaagagttccagaccacagatattccggtgcatcactgtaacttccgggctgttctcggctgcctttgtagcgcttctgttctcggtagctacgcagggccagcaccacgctggcgccgtacatgatcacgagaagacaagcaaaggtggctgctgctccgtcggtgcctgccagctggcagtccatccaggtgagacccttgcgggcatagagcctctctcttgttttgcaagtgtcggtgctattgatctgcagagccacgtggaggtaaacaccaatgcctgtgcagtagcccactgccgctaggaggctgaaggcggcctccgtgaggagccacttccctgacaacattgttcgactcttggctccttggagtaaaacacccatggtgaggacccccagacccagagaaacagccacgccaccgtatatcaggggcgagcggaggatcgtgtactgctggtccagctgccgaacctgctctagctcagtgccctcgaacggtgagtagtagttgttcccaaagccaccgccgctggaaaagctggcactgaatccggcaaggacaaagtaggaggccacgatgcatatgagaaccatcccattcaagaccacctccactatctgcaccacacctctcccagtgcacaagtatttgcatttgtggcattccaggagtccttccgcctctgactggtaatattccacctcctctcgtccaggcctgggggtcgagggcagatatctctccgaagggggttcactttcgggtctgcggcgcccggggtctcccttcctctgcggctgcggcggctccggggcttcccagggcgcgggcccaggaggcgcggctgcgtcccaggtcagtccccgggctccgtcccgcgtccggctttggcgcggtttttcccaaactccgtgttcacctgcgcgagggcccgcgtccctgtgtgtgtcccggcgggggcctcggtccgggtctctttccctctctctctccctctcccggtcccggttccggtcgcggttcccgtccctctcctggtctctctccgggtcccggtccccgtcccttcgccggttcccgtcgctgcttcgcttcctgcgcgggtccccgggtcggtcccgcggtcgatcgtgggtgcggccttggtctgggtgggggcgccgtcccgggtcccgctctctcggccgggcccggggctcgcgagcccccgacggatcttccatggccgggttccgtgtccccgcccgggagcgacctgagggcaacaac

SEQ ID NO: 13793 - RNA, 2259 nt, Homo sapiens
  source 1..2259: mol_type = other RNA
gctgggattacaggcatgagccaccatgcccgtctaattttgtatttttagtagagacggggtttctccatattaagtcaggctggtctcgaactcccgacctcaggtgatcctcccgcctcagcctcccaaagtgctgggattacaggcgtgagccacggcgcccggccctgccatttctacttatttacgttgttccaaattatcaaagatagcatcaactttcaaatcctaattttttttttcctgggaaaccttcctcctttagccttcagtctcctctctaaactgggttgggcctcagttcttctcataccgggtctccccttcctgctgtcctgggttgtatcttccgcttcctagatttaaggtctttatttttcagccaagatgggtcatcctcatggctggtggcattggactgtaaatactagttgccttcatccccacatttggaatatacctgcaatcatacaggatgcagaatactgtttgctaagcgtggggctggttgctggagataacaagcaaggcctaccaggtccctgctgtcattctggctctggatctacttgcttggctcccctgccagccctagtatatcgagccttcctttttattcaatagtgttttttattgctgacttttcagtcaagatttctttgtgttttctggcctacccttgctgtttttcacctgaaatgctttttggcttttagtgtgactcctgctgatctcatatgcatatgttattaattgattaattattaattgttaataattaaatattattaatatgcttacattattaccttgagttctggaactgcctcactgcactccatgtggtgaatactcttttgttcattccttcaaaagtttcctcttcaaaagtagggctagcagatcttgcctcttcctctccagggaaacgctgaccagtttgtgtgaacgccatcacccacactcttgaaatatatctggaaagtgccggaagtgaactgggggatccttgcctcccaaaacagggatgggctctgaacgccccaccacggcctgctgccacgcgcgcctctcgctgcaggagcggtggatccaccgatgggcttccagggcggtcttgcgcttgaagcctttcccacactccacgcaggggaagggccggctgtcggagtgaatgcgccggtgactgaggaggagggaagaataggtgaagcggcggccgcagtcaggacaggggtagggcttctcgccggtgtgtatgcgcctgtggatggccagcagggaggtgtaggcgaaacggaggctgcaatcggggcagctgtagggcttctcgcccgtgtgcttgcgctggtggatggccagcaggtaggggtaagtgaagcgactcttgcagtctgagcacgcgtaaggcttctccccggtgtgagcccgcctgtggatagccagggaacccctctggcggaagcggcgcccgcagtcggggcaggggtagggcttctcgccggtgtggatgaactgatgctggagcaggtacctgcgctgggagaaacgcgcctgacactggccgcaggagaagggccgctccccggagtggacccgctggtggctggccaggagggaagggtagctgaagttgcggccacagtctgggcaagagtggggcagtcttcgggtcagagtgtccttgagccagggattcatggggctctgcctagggttgcagaactctgggcaggcgacgctgggccaccactccttgacagccacttcatgcgccacctctttttgttttggacacttcttcagcctttccttctcctcattcccatccctggatcctgcttcctgtccttggcccctgctgaaagctgcagagctctcaccgtcgggatcctgggcctccgggctccacgcctccacttctccttccacccacgagataaaagcgggtttgggaactgaaaatcccagcgcgcccaggtggccgaaggtctcccgcatcacgtcccggtacagggccctctgcgctggccgcaggcattcccactcctcgggagagaagtacacggccacgtccgcgaagctcacggcgcccggcctgctttccctcgtcctccggggcccggcctccccgggtacgtgggccgggcgcggcgccaggggcggccccatgggaaaccctttctgcctggcaaagggaggcttccggggaaggtggagatgctggcgctttcctgtctttcctcagacaagtcc

SEQ ID NO: 13794 - RNA, 2641 nt, Homo sapiens
  source 1..2641: mol_type = other RNA
gctgggattacaggcatgagccaccatgcccgtctaattttgtatttttagtagagacggggtttctccatattaagtcaggctggtctcgaactcccgacctcaggtgatcctcccgcctcagcctcccaaagtgctgggattacaggcgtgagccacggcgcccggccctgccatttctacttatttacgttgttccaaattatcaaagatagcatcaactttcaaatcctaattttttttttcctgggaaaccttcctcctttagccttcagtctcctctctaaactgggttgggcctcagttcttctcataccgggtctccccttcctgctgtcctgggttgtatcttccgcttcctagatttaaggtctttatttttcagccaagatgggtcatcctcatggctggtggcattggactgtaaatactagttgccttcatccccacatttggaatatacctgcaatcatacaggatgcagaatactgtttgctaagcgtggggctggttgctggagataacaagcaaggcctaccaggtccctgctgtcattctggctctggatctacttgcttggctcccctgccagccctagtatatcgagccttcctttttattcaatagtgttttttattgctgacttttcagtcaagatttctttgtgttttctggcctacccttgctgtttttcacctgaaatgctttttggcttttagtgtgactcctgctgatctcatatgcatatgttattaattgattaattattaattgttaataattaaatattattaatatgcttacattattaccttgagttctggaactgcctcactgcactccatgtggtgaatactcttttgttcattccttcaaaagtttcctcttcaaaagtagggctagcagatcttgcctcttcctctccagggaaacgctgaccagtttgtgtgaacgccatcacccacactcttgaaatatatctggaaagtgccggaagtgaactgggggatccttgcctcccaaaacagggatgggctctgaacgccccaccacggcctgctgccacgcgcgcctctcgctgcaggagcggtggatccaccgatgggcttccagggcggtcttgcgcttgaagcctttcccacactccacgcaggggaagggccggctgtcggagtgaatgcgccggtgactgaggaggagggaagaataggtgaagcggcggccgcagtcaggacaggggtagggcttctcgccggtgtgtatgcgcctgtggatggccagcagggaggtgtaggcgaaacggaggctgcaatcggggcagctgtagggcttctcgcccgtgtgcttgcgctggtggatggccagcaggtaggggtaagtgaagcgactcttgcagtctgagcacgcgtaaggcttctccccggtgtgagcccgcctgtggatagccagggaacccctctggcggaagcggcgcccgcagtcggggcaggggtagggcttctcgccggtgtggatgaactgatgctggagcaggtacctgcgctgggagaaacgcgcctgacactggccgcaggagaagggccgctccccggagtggacccgctggtggctggccaggagggaagggtagctgaagttgcggccacagtctgggcaagagtggggcagtcttcgggtcagagtgtccttgagccagggattcatggggctctgcctagggttgcagaactctgggcaggcgacgctgggccaccactccttgacagccacttcatgcgccacctctttttgttttggacacttcttcagcctttccttctcctcattcccatccctggatcctgcttcctgtccttggcccctgctgaaagctgcagagctctcaccgtcgggatcctgggcctccgggctccacgcctccacttctccttccacccacgagataaaagcgggtttgggaactgaaaatccgacggactgggggtcccggccggagggcccggcctcacccagcgcgcccaggtggccgaaggtctcccgcatcacgtcccggtacagggccctctgcgctggccgcaggcattcccactcctcgggagagaagtacacggccacgtccgcgaagctcacggcgcccggcctgctttccctcgtcctccggggcccggcctccccgggtacgtgggccgggcgcggcgccaggggcggccccatgggaaaccctttctgcctggcaaagggaggcttccggggaaggtggagatgctggcgctttcctgtctttcctcagacaagtccgtaagggactcctgcccttaaccaagatggaaccttcctggcgtcaacacccctcgcctttcctctctgcctttacacaccacgagggaaaccagcgggaagggtggccccgcaacaccactaaccgatagatggcgtacgttgattggacagtgccggaaggccaggagaagaaggaaggctgtgattgggcttttttttggagtggcctgtttgaaaggctgagggtgaaggagcgacagatctgaaaatagccggagctgaggggcctcagggtctaccctgactcgcttttcccggacggtctcctaggagagaggctgtggccagctgacgcgacttc

SEQ ID NO: 13795 - RNA, 2206 nt, Homo sapiens
  source 1..2206: mol_type = other RNA
gctgggattacaggcatgagccaccatgcccgtctaattttgtatttttagtagagacggggtttctccatattaagtcaggctggtctcgaactcccgacctcaggtgatcctcccgcctcagcctcccaaagtgctgggattacaggcgtgagccacggcgcccggccctgccatttctacttatttacgttgttccaaattatcaaagatagcatcaactttcaaatcctaattttttttttcctgggaaaccttcctcctttagccttcagtctcctctctaaactgggttgggcctcagttcttctcataccgggtctccccttcctgctgtcctgggttgtatcttccgcttcctagatttaaggtctttatttttcagccaagatgggtcatcctcatggctggtggcattggactgtaaatactagttgccttcatccccacatttggaatatacctgcaatcatacaggatgcagaatactgtttgctaagcgtggggctggttgctggagataacaagcaaggcctaccaggtccctgctgtcattctggctctggatctacttgcttggctcccctgccagccctagtatatcgagccttcctttttattcaatagtgttttttattgctgacttttcagtcaagatttctttgtgttttctggcctacccttgctgtttttcacctgaaatgctttttggcttttagtgtgactcctgctgatctcatatgcatatgttattaattgattaattattaattgttaataattaaatattattaatatgcttacattattaccttgagttctggaactgcctcactgcactccatgtggtgaatacttgcctcttcctctccagggaaacgctgaccagtttgtgtgaacgccatcacccacactcttgaaatatatctggaaagtgccggaagtgaactgggggatccttgcctcccaaaacagggatgggctctgaacgccccaccacggcctgctgccacgcgcgcctctcgctgcaggagcggtggatccaccgatgggcttccagggcggtcttgcgcttgaagcctttcccacactccacgcaggggaagggccggctgtcggagtgaatgcgccggtgactgaggaggagggaagaataggtgaagcggcggccgcagtcaggacaggggtagggcttctcgccggtgtgtatgcgcctgtggatggccagcagggaggtgtaggcgaaacggaggctgcaatcggggcagctgtagggcttctcgcccgtgtgcttgcgctggtggatggccagcaggtaggggtaagtgaagcgactcttgcagtctgagcacgcgtaaggcttctccccggtgtgagcccgcctgtggatagccagggaacccctctggcggaagcggcgcccgcagtcggggcaggggtagggcttctcgccggtgtggatgaactgatgctggagcaggtacctgcgctgggagaaacgcgcctgacactggccgcaggagaagggccgctccccggagtggacccgctggtggctggccaggagggaagggtagctgaagttgcggccacagtctgggcaagagtggggcagtcttcgggtcagagtgtccttgagccagggattcatggggctctgcctagggttgcagaactctgggcaggcgacgctgggccaccactccttgacagccacttcatgcgccacctctttttgttttggacacttcttcagcctttccttctcctcattcccatccctggatcctgcttcctgtccttggcccctgctgaaagctgcagagctctcaccgtcgggatcctgggcctccgggctccacgcctccacttctccttccacccacgagataaaagcgggtttgggaactgaaaatcccagcgcgcccaggtggccgaaggtctcccgcatcacgtcccggtacagggccctctgcgctggccgcaggcattcccactcctcgggagagaagtacacggccacgtccgcgaagctcacggcgcccggcctgctttccctcgtcctccggggcccggcctccccgggtacgtgggccgggcgcggcgccaggggcggccccatgggaaaccctttctgcctggcaaagggaggcttccggggaaggtggagatgctggcgctttcctgtctttcctcagacaagtcc

SEQ ID NO: 13796 - RNA, 2588 nt, Homo sapiens
  source 1..2588: mol_type = other RNA
gctgggattacaggcatgagccaccatgcccgtctaattttgtatttttagtagagacggggtttctccatattaagtcaggctggtctcgaactcccgacctcaggtgatcctcccgcctcagcctcccaaagtgctgggattacaggcgtgagccacggcgcccggccctgccatttctacttatttacgttgttccaaattatcaaagatagcatcaactttcaaatcctaattttttttttcctgggaaaccttcctcctttagccttcagtctcctctctaaactgggttgggcctcagttcttctcataccgggtctccccttcctgctgtcctgggttgtatcttccgcttcctagatttaaggtctttatttttcagccaagatgggtcatcctcatggctggtggcattggactgtaaatactagttgccttcatccccacatttggaatatacctgcaatcatacaggatgcagaatactgtttgctaagcgtggggctggttgctggagataacaagcaaggcctaccaggtccctgctgtcattctggctctggatctacttgcttggctcccctgccagccctagtatatcgagccttcctttttattcaatagtgttttttattgctgacttttcagtcaagatttctttgtgttttctggcctacccttgctgtttttcacctgaaatgctttttggcttttagtgtgactcctgctgatctcatatgcatatgttattaattgattaattattaattgttaataattaaatattattaatatgcttacattattaccttgagttctggaactgcctcactgcactccatgtggtgaatacttgcctcttcctctccagggaaacgctgaccagtttgtgtgaacgccatcacccacactcttgaaatatatctggaaagtgccggaagtgaactgggggatccttgcctcccaaaacagggatgggctctgaacgccccaccacggcctgctgccacgcgcgcctctcgctgcaggagcggtggatccaccgatgggcttccagggcggtcttgcgcttgaagcctttcccacactccacgcaggggaagggccggctgtcggagtgaatgcgccggtgactgaggaggagggaagaataggtgaagcggcggccgcagtcaggacaggggtagggcttctcgccggtgtgtatgcgcctgtggatggccagcagggaggtgtaggcgaaacggaggctgcaatcggggcagctgtagggcttctcgcccgtgtgcttgcgctggtggatggccagcaggtaggggtaagtgaagcgactcttgcagtctgagcacgcgtaaggcttctccccggtgtgagcccgcctgtggatagccagggaacccctctggcggaagcggcgcccgcagtcggggcaggggtagggcttctcgccggtgtggatgaactgatgctggagcaggtacctgcgctgggagaaacgcgcctgacactggccgcaggagaagggccgctccccggagtggacccgctggtggctggccaggagggaagggtagctgaagttgcggccacagtctgggcaagagtggggcagtcttcgggtcagagtgtccttgagccagggattcatggggctctgcctagggttgcagaactctgggcaggcgacgctgggccaccactccttgacagccacttcatgcgccacctctttttgttttggacacttcttcagcctttccttctcctcattcccatccctggatcctgcttcctgtccttggcccctgctgaaagctgcagagctctcaccgtcgggatcctgggcctccgggctccacgcctccacttctccttccacccacgagataaaagcgggtttgggaactgaaaatccgacggactgggggtcccggccggagggcccggcctcacccagcgcgcccaggtggccgaaggtctcccgcatcacgtcccggtacagggccctctgcgctggccgcaggcattcccactcctcgggagagaagtacacggccacgtccgcgaagctcacggcgcccggcctgctttccctcgtcctccggggcccggcctccccgggtacgtgggccgggcgcggcgccaggggcggccccatgggaaaccctttctgcctggcaaagggaggcttccggggaaggtggagatgctggcgctttcctgtctttcctcagacaagtccgtaagggactcctgcccttaaccaagatggaaccttcctggcgtcaacacccctcgcctttcctctctgcctttacacaccacgagggaaaccagcgggaagggtggccccgcaacaccactaaccgatagatggcgtacgttgattggacagtgccggaaggccaggagaagaaggaaggctgtgattgggcttttttttggagtggcctgtttgaaaggctgagggtgaaggagcgacagatctgaaaatagccggagctgaggggcctcagggtctaccctgactcgcttttcccggacggtctcctaggagagaggctgtggccagctgacgcgacttc

SEQ ID NO: 13797 - RNA, 3257 nt, Homo sapiens
  source 1..3257: mol_type = other RNA
gctgggattacaggcatgagccaccatgccctgcccccactttttctttaaaaatggtaaccctttacactcttctgcacattaagaacagctagacctaagtttaagcacagtactagcttgatgacttgtgatcctccctgaacctgtttcctcctctaaaatggcagtaatagcaagacacctcactgttgtcggggagtgccaggagagaatgcttgctgcgaagctgtcagcacacggcctggaatagagtgagtgctccatatctggaagttatgattaattctgcatcctagggtggccaggcggggcttcccagtgccagaggtacagactgagaaccacacccttggtgaggccaccctacttatgacttagggggcagagagaacctcagtaaggtcagtggtgtttattgaggctttactatgtgctatgtgcctcttgctgaggtcttagctagaatcgtggtatttcagggtttctcaacattttttttttttttttttttggagatggtgtctcgctctgtcgcccaggctggagtgcaatggcgcaatctcggctcactgcaacctctgccacccaggttcaagcaattctcctgcctcagcctcccaagtagttgggattacaggtgctgaattcttttttttttttttttttgtagcatggtgatattgcactatgcttaaccgcatccctggtctctactcactcaatgccagtagccttcttcctgcctgttgtgacatcaaaaatgtcatacattgccaaatgtccccaagaaagagtggggctgagggaggacaaaatcctacccacagtttaaaaccaccgccttatctcatcctcacagtaactaaccacagtaaccccaggtggtaagtactgttaatgccccatattgcaagtgaggagaccaacagaacagagtttgggtgacattcctgagaacacacagctccgagattcacgcccaggcactgtgactccagagctcacctgcccattatgcaagaacatctgatcttggctgggagcagtggctcacacctgtaatcccagcactttgggagtccaaggcgggcagatcacgaggtcaggagatcgagaccgtcctggccaacatggtgaaaccctgtctctactaaaaatacaaaaaattagccttggtggcaggtgcctgtaatcccagctacttgggaggctgaggcaggataatcgcttgaaccagggaggcgaggttgcagtgagccgagattgtgccactgcactccagcctgggtgacagagcaagactctgtctcaaaaaaaaaaaaaaaaaaaaaaaaaaggccaggctcgatggctcacacctgtaatcccagcactttaggagactgagcggggcagatcacgaggtcaggagttcaagaccagcctgaccaacatggtgataccccatctctactaaaaatacaaaaattagctgggctcagtggcatgcgcctgtaatcccagctactcaggaggctgaggtaggagaatcgcttgaacatgggaggcagaggttgcagtgagctgagatcgcgccactgcattccagcctgggcaatagagggagactacgtcttaaaaaaaaaaaatcacctggggaattttctgaaagctcaggcctcaccccagatgaattagatgtgaacctgtgaatctctgggcatgggacctgggcttccacagctttgcaaagtttccatgggatttcaaggttgagagccctgtgttaggctgagaagtggtcaggaaattttatgatctccaatcttggcagccagtgtggcaggatacaggccttctctctgggtcatctgggttatctcacaggggacctgccatttctttctctttttcttttcctttcttttatattttaaaatttttttttgtagagtcagggtcttgctatgttgcctaagctggtctcgaactcctggcctcaggcagtcctcttaccttggcctcccaagttctgggattacaggaatgagccactgcacccggcctaagacctgcccttactcccccaagctaaacccaggcagcccagccaaggcaggtcttccctcttctaaacctgaaagccctgctgagccccctcgagtgccccatccttatcccataggcccaggcttataccacttggttattctttattctcatgcattccaggatgagatcagagaatgaagagggtcccgaggacagcctgggagagaagcaccagccttcctattggcaagaaatgacccagtgctgggggtagtgaggggccctatgagggtgccggggtcatgcctggagctgctgctgactcctccagccagagccgcactggtctgagcgatcgggtgacacaggcttgaatttctcctgaagcgtttgtgttctctggcatcaatctccttcctctgtcttcctgaacatggccaaggcctccgccagcacaccatcagggtctaggattttgacctcaggaatggggaactgagtgggctcaggggcctcgtcacggccaaagtcgatcatcgtcccgcatttggccatattgtccacccagaagccttcaaacagctggccgtggtccagatggaagaaacgccccgccccgttcttcatgcctctctcccagcagccctcgtagcggttcccgttcttcaggcgcagcatgccctccccgttgggcttgtcgttctcccactgtccctcgtagatgtcgccgttgctgtaatacatgcggccccacccgctgcgctggctgccacaccagtcaccctcataatactccttgggtccgaaaaactggatcccataacccgatttcttatcacctttccaccagcctgagtagactctcctgcactttcctgtctgttggtcaggaaggctgagggtgccgtagccgtctcgcttcccaaacttccagtccccctcatagatggctcctttcttcttccagacctgtgttcctttcccgtgtttcacgttgtccttccactcgcccacatagtagtcgccattcacagcgtatacctggctccgcaggccgttcctctgggccttccggtcccaccccttccacagggactccgacttttttgggcacttagagactggcatggtggctgcttctgcaaggctggagggtgctgcgggatcgcagcatccagcctcaatgtccgtcagctgcgcgcgccgcgggcccggccggggtc

SEQ ID NO: 13798 - RNA, 3333 nt, Homo sapiens
  source 1..3333: mol_type = other RNA
gctgggattacaggcatgagccaccatgccctgcccccactttttctttaaaaatggtaaccctttacactcttctgcacattaagaacagctagacctaagtttaagcacagtactagcttgatgacttgtgatcctccctgaacctgtttcctcctctaaaatggcagtaatagcaagacacctcactgttgtcggggagtgccaggagagaatgcttgctgcgaagctgtcagcacacggcctggaatagagtgagtgctccatatctggaagttatgattaattctgcatcctagggtggccaggcggggcttcccagtgccagaggtacagactgagaaccacacccttggtgaggccaccctacttatgacttagggggcagagagaacctcagtaaggtcagtggtgtttattgaggctttactatgtgctatgtgcctcttgctgaggtcttagctagaatcgtggtatttcagggtttctcaacattttttttttttttttttttggagatggtgtctcgctctgtcgcccaggctggagtgcaatggcgcaatctcggctcactgcaacctctgccacccaggttcaagcaattctcctgcctcagcctcccaagtagttgggattacaggtgctgaattcttttttttttttttttttgtagcatggtgatattgcactatgcttaaccgcatccctggtctctactcactcaatgccagtagccttcttcctgcctgttgtgacatcaaaaatgtcatacattgccaaatgtccccaagaaagagtggggctgagggaggacaaaatcctacccacagtttaaaaccaccgccttatctcatcctcacagtaactaaccacagtaaccccaggtggtaagtactgttaatgccccatattgcaagtgaggagaccaacagaacagagtttgggtgacattcctgagaacacacagctccgagattcacgcccaggcactgtgactccagagctcacctgcccattatgcaagaacatctgatcttggctgggagcagtggctcacacctgtaatcccagcactttgggagtccaaggcgggcagatcacgaggtcaggagatcgagaccgtcctggccaacatggtgaaaccctgtctctactaaaaatacaaaaaattagccttggtggcaggtgcctgtaatcccagctacttgggaggctgaggcaggataatcgcttgaaccagggaggcgaggttgcagtgagccgagattgtgccactgcactccagcctgggtgacagagcaagactctgtctcaaaaaaaaaaaaaaaaaaaaaaaaaaggccaggctcgatggctcacacctgtaatcccagcactttaggagactgagcggggcagatcacgaggtcaggagttcaagaccagcctgaccaacatggtgataccccatctctactaaaaatacaaaaattagctgggctcagtggcatgcgcctgtaatcccagctactcaggaggctgaggtaggagaatcgcttgaacatgggaggcagaggttgcagtgagctgagatcgcgccactgcattccagcctgggcaatagagggagactacgtcttaaaaaaaaaaaatcacctggggaattttctgaaagctcaggcctcaccccagatgaattagatgtgaacctgtgaatctctgggcatgggacctgggcttccacagctttgcaaagtttccatgggatttcaaggttgagagccctgtgttaggctgagaagtggtcaggaaattttatgatctccaatcttggcagccagtgtggcaggatacaggccttctctctgggtcatctgggttatctcacaggggacctgccatttctttctctttttcttttcctttcttttatattttaaaatttttttttgtagagtcagggtcttgctatgttgcctaagctggtctcgaactcctggcctcaggcagtcctcttaccttggcctcccaagttctgggattacaggaatgagccactgcacccggcctaagacctgcccttactcccccaagctaaacccaggcagcccagccaaggcaggtcttccctcttctaaacctgaaagccctgctgagccccctcgagtgccccatccttatcccataggcccaggcttataccacttggttattctttattctcatgcattccaggatgagatcagagaatgaagagggtcccgaggacagcctgggagagaagcaccagccttcctattggcaagaaatgacccagtgctgggggtagtgaggggccctatgagggtgccggggtcatgcctggagctgctgctgactcctccagccagagccgcactggtctgagcgatcgggtgacacaggcttgaatttctcctgaagcgtttgtgttctctggcatcaatctccttcctctgtcttcctgaacatggccaaggcctccgccagcacaccatcagggtctaggattttgacctcaggaatggggaactgagtgggctcaggggcctcgtcacggccaaagtcgatcatcgtcccgcatttggccatattgtccacccagaagccttcaaacagctggccgtggtccagatggaagaaacgccccgccccgttcttcatgcctctctcccagcagccctcgtagcggttcccgttcttcaggcgcagcatgccctccccgttgggcttgtcgttctcccactgtccctcgtagatgtcgccgttgctgtaatacatgcggccccacccgctgcgctggctgccacaccagtcaccctcataatactccttgggtccgaaaaactggatcccataacccgatttcttatcacctttccaccagcctgagtagactctcctgcactttcctgtctgttggtcaggaaggctgagggtgccgtagccgtctcgcttcccaaacttccagtccccctcatagatggctcctttcttcttccagacctgtgttcctttcccgtgtttcacgttgtccttccactcgcccacatagtagtcgccattcacagcgtatacctggctccgcaggccgttcctctgggccttccggtcccaccccttccacagggactccgacttttttgggcacttagagactggcatggtggctgcttctgcaaggctggagggtgctggaaaggggttagggacatctggggctcagcgcgccccgtgtaatgccgggatcctgagctcaagtggggagagtcatgtgtgttctgagtccctggggcaggtgaacagcccttagtggggatcctttagtgctggact

SEQ ID NO: 13799 - RNA, 70 nt, Homo sapiens
  source 1..70: mol_type = other RNA
gctgggattacaggcatgagccaccatgccctgcctgttgtgtcatctgtctgtctgtctgtctgtctgt

SEQ ID NO: 13800 - RNA, 1883 nt, Homo sapiens
  source 1..1883: mol_type = other RNA
gctgggattacaggcatgagccaccatgccctgctgaattttcctatgtttagtaagagttgaggattggttaaaggctttaccacattcttcacatttgtaagatttctctccagtatgaattatgttatgtttagtaaggtttgaggatcggttgaaagctttgccacattcttcacatttgtagggtttctctccagtgtgaattctcttatgtgtagtaaggtttgaggatcggttaaaagctttgccacattcttcacatttgtagagtttctctccagtatgaattatcttatgtttggtaaggtttgaggattggttaaaagctttgccacattcttcacatttgtaaggtttctctccagtatgaattatcttatgtatagtaagttttgaggagtggttaaaggctttgccacattcttcacatttgtagggtttctctccagtatgaatcatcttatgtgtagtaaggtgtgaagacacattaaaggctttgccacattcttcacatttgtagggtttctctccagtatgaattcttttatgttttgtaagggttgaagaccagttaaagcctttgccacattgttcacatttgtaagatttctctccagaatgaattatcttatgtttagtaaggtatgagaatcggttaaaagctttgtcacattcttcacatttgtagggtttttctttaacatgaatgaacttatgtgtagtaagggctgaagggtggttaaaagctttaccacattcttcacatttgaagggcttctctccagtatgaattaccttatgtgtagtaaggtgtgaagaatggtagaaggctttgccacattcttcacatctgtagggtttctctccagtatgaatcatcttatgtgtagtaagggttgaggagtgcttaaaagctttgccacattcttcacatttgaagggtttctctccagtatgaactctcttgtgtctagtaagggttgagaaccgcttaaacactttgtcacattcttcacattggtaagaattctctctaatatgaattcttttatgttgatgtaggtgtaaaagcatgcaaaatgattcatcacattttttacatttgaaaggtttctctccagtatgtcttgtcttgtgtctatttgaattgaaaattttatgaaagacttttatatatttatcacatggaaatattttgctctgggtagttgtcaaacactggtttagttcattataaccttttttgtacaccttacactcaaccacatttgcggagccttttcttaactgtaaattctcatgttcacatttgccatgtcttctcagtatcacttgttgaaaagaatcttttatgtcttgctctggccaaaggtctctggtaaaagaagaacacatagctgcacatcctgcacatgtatcctggggattcatccaccatctcacatatcttcatattccagggctctttttcttgctctagactggtgatcgggtcttgcttagagacagcaatacccaagaagaccaggtttttgtagttctctaacatcacattcatatataaattctgctgagcagggttcaggcattcccactcctccagagagaattctatggccacatccctaaatgtcaacgtctccttttcaaagtaagagtacactagaagcttcctctctgccccagggatccacttgctcccttgagaggatacactccagacctcaggtcgcccatttctaggcttccggggtacctggcgtcttagctgtggatctctcaatacctgcaggtcacagggccacagaggctgggcctctgcgagcagaggacacagggcagtgaaggcgagacctgcagctccagctgcagcgagagac

SEQ ID NO: 13801 - RNA, 1864 nt, Homo sapiens
  source 1..1864: mol_type = other RNA
gctgggattacaggcatgagccaccatgccctgctgaattttcctatgtttagtaagagttgaggattggttaaaggctttaccacattcttcacatttgtaagatttctctccagtatgaattatgttatgtttagtaaggtttgaggatcggttgaaagctttgccacattcttcacatttgtagggtttctctccagtgtgaattctcttatgtgtagtaaggtttgaggatcggttaaaagctttgccacattcttcacatttgtagagtttctctccagtatgaattatcttatgtttggtaaggtttgaggattggttaaaagctttgccacattcttcacatttgtaaggtttctctccagtatgaattatcttatgtatagtaagttttgaggagtggttaaaggctttgccacattcttcacatttgtagggtttctctccagtatgaatcatcttatgtgtagtaaggtgtgaagacacattaaaggctttgccacattcttcacatttgtagggtttctctccagtatgaattcttttatgttttgtaagggttgaagaccagttaaagcctttgccacattgttcacatttgtaagatttctctccagaatgaattatcttatgtttagtaaggtatgagaatcggttaaaagctttgtcacattcttcacatttgtagggtttttctttaacatgaatgaacttatgtgtagtaagggctgaagggtggttaaaagctttaccacattcttcacatttgaagggcttctctccagtatgaattaccttatgtgtagtaaggtgtgaagaatggtagaaggctttgccacattcttcacatctgtagggtttctctccagtatgaatcatcttatgtgtagtaagggttgaggagtgcttaaaagctttgccacattcttcacatttgaagggtttctctccagtatgaactctcttgtgtctagtaagggttgagaaccgcttaaacactttgtcacattcttcacattggtaagaattctctctaatatgaattcttttatgttgatgtaggtgtaaaagcatgcaaaatgattcatcacattttttacatttgaaaggtttctctccagtatgtcttgtcttgtgtctatttgaattgaaaattttatgaaagacttttatatatttatcacatggaaatattttgctctgggtagttgtcaaacactggtttagttcattataaccttttttgtacaccttacactcaaccacatttgcggagccttttcttaactgtaaattctcatgttcacatttgccatgtcttctcagtatcacttgttgaaaagaatcttttatgtcttgctctggccaaaggtctctggtaaaagaagaacacatagctggggattcatccaccatctcacatatcttcatattccagggctctttttcttgctctagactggtgatcgggtcttgcttagagacagcaatacctgccaagaagaccaggtttttgtagttctctaacatcacattcatatataaattctgctgagcagggttcaggcattcccactcctccagagagaattctatggccacatccctaaatgtcaacgtctccttttcaaagtaagagtacactagaagcttcctctctgccccagggatccacttgctcccttgagaggatacactccagacctcaggtcgcccatttctaggcttccggggtacctggcgtcttagctgtggatctctcaatacctgcaggtcacagggccacagaggctgggcctctgcgagcagaggacacagggcagtgaaggcgagacctgcagctccagctgcagcgagagac

SEQ ID NO: 13802 - RNA, 6117 nt, Homo sapiens
  source 1..6117: mol_type = other RNA
gctgggattacaggcatgagccaccatgccctgtgcctcacgttatttctttgtactgaacatcttcagtgagtaactgatccctcatatagtgaattattcttccaaatgagtgcatttcctgtgctaactatgatagcttgtagagttgatggatttaggtttcaacatgttatgggagtctactaccggaagagaggaaaaagctttgcttcaggaagattttaggagttttgagattctgctgtgaattttggaaaggtttagccttaaaaacatttggtggtaaccttagaagcctggtatctgtagaccacctgtcaggcccaacagtgggctgtttttctattagtccctacttgggagaaaagccaagtagtattgtcagtgcccttgctgtccagaaacctgtgatctacctaagtgcagagagcaccttgccagtgtacacaagcaaatgctgaccacattctagtctcttgctaccaagtatggtcccaggaccagcagcaccaagcctcactccagggctaccaagttggaatcttcagtctaatgaaatgtggatagtttgcgtgcagatttaatgtttgagaagcaccgtccatgagtgcttggtggttctccacctttcaaagctacaaactcatttgaaaatctcatgggatttatgagcacccttggaaaagcatattgattgatacacaaaatttttcatatgcagtttcagagttcctgtaaataatctattgatgccagggaagtcctaggttaagaccccctagtcacaaagaagattgactcagtgtcagctggaggagttaagagaagattctcacagggggcagagcttaaattaaacctggggaatttgataggaagaggagtaaagaagagcatttcaagctgttgaaatgcaaaggtcctgagagggaaaaagagaatgtccttttttgtatgtgttcatgtgaaacttaatgaggagattgttgtttgacagcaggctttccttgcaattccttatcatcacttgaacgtccagaaaatgaagccagactgtggactcagtagtcattccactttgggtgtgcaagaaccctatgacatgggggtttcacataagatctcatttcctactactttgctcacctctcactctgccccagccacattggccttcaggctgttccaggcactcccgacaacagagcctggcccactcttgtctgtgtggggattcttccccaaatcagcaaaaggctcattaagatctttattcaaatgagacttcaagggagaggctttctttctaaaatagcagcccctcccacactccctttccctaaataaaacaggaagaacaattgcttcactacttgcgttatatttatttacaaattcatttatggcctgtttccttaaatgtatgaactttatttgctgctgtatctcctgtgcctagaatagggcctggcatatagtaggtactcaataaatgtttattgaataaatgatcttttaactacaaccagtaatgagtgtaaaagccatgtttacaactctatagctacgaaatcataatatatgaaacattcttggaatataccacatgtttgctgagactgaattttcaaccacttctctttagtctaatgaaacaagaaacactaaacacatggaacattttaagtttgaaaattcaaacattttaaagtaagacttacaaaaaatgtctgtatagtccatgtataatgcacaactatttttcttctggcaaagctgagacacattcatgtgtactcagctggggttttcttccaaaatgccacatccaggctgaattcatgtgtgtatggtctggattatccccctaagttagatttaaggaaaatgtaggagaagctggaaggttagaacattttgaatgagaatttccttaaagcttgagtattctcctccttactacccaattaaaatttcaccagtcctggaaatatgtcaacctctgctaatgaacttgattgactaattgccaaggctaaggaattttctaaccagtgatttccttgtaaataaagaaatttaggtcacatcttggttgggagatttcagctttgcctaatcaaatgcagcaggaaatggtatactatgagatatactatgagaggctatgtttgcatgaggactacaggcctagggtacagttctaagcaggttacacggtcactcaccataaccaccaaatacgtttttggcatttgtattagctcttgaacttgggccagcaccaatttaatttgtgcataagaccttcaaatatagatgcatacttgatcctgttagtgtaaaccagtgactaataaagagcattactgtatatttatatagccttctatacttctaaaaacactttttcatttcatcttcattttaggtcgttctgttcttgctgggtaggtaaggcatttatggttgatttacacatttcttctttccagaagggatttgaggcaaagtagaaggcttttgtatagaatgagtcattccttttttttccagctttactgaggtataattgattgagtcatgcctattgtactctttgttatgtgttctttccccacatacctgtatgtctccctccttagctttcttcccatgtctgcttaaatctgaactcccagaggcctgccttccaagacatcctagataaagtatcacccatggccttccttatcccagtaccccctttattcttctacatagcacttaacacctgacatgttgattgtatatttatttgtttattgcctccctgctccccataccactagaatataaactccatgaggggcagaaatattgcctattttattcatggctgtatcccaaccccgtgatcagtgcttggcacatagtagagatttaataaatatttgttgaatgaataaatgaatgaagccccagtgcttagggcaggcgcctgtcatgtgataaatatttgttgaattaaacaaagctttaatgaatgagctagagaaaggtctgtgattcattcaaggttatgcagacagtgataacttgctttatctagatgcgaatccccgctaattctttctccaagccttcttcatttgtatacctcgtagcaaatccagcctgttgtaatgtcagaatgtctttgttcatcctttttggtacctgtaatcccagcactttcggaggtggaggcaggtagatcacaaggccaagatggtgcaaccctgtccctcaagcatctggagaagcttatactgctcagatctcaggaaccagggaggtcacgggggaaaagaccaaggacagtcgcaggcagcttcagcaaaagtagacccaacaataaaaatgatgtaagaagtgtattaagtatgtctttttattctgattcttcaacatcttggagtctagctgacgttgaaaggaactgcccctcccagggttatgaaattcctagagatagcaacttgcctgggagcctatctttcatacgcaaaccagccaatccaaagcccacacttctaccacctcctttatctggctcttatatgcagacccactatcccactgtcctaatcaccctaggccatgacaggataccagatgactagagacagcccctatgccccagatcctgctggaattattcaaactagccaatcctaaacctgcttactctgcctttcccttctcaataaaggttcttgtccacgatcccccctcactccttctttctcttgactcacccttctccatgttgccctacctagggtgctcctgttattaggtatctgtaagtataaaaacttattccttcatgactgtcttttctgcatgtcttaccatacctgattaaaacaaatcccaggtactcttatattaataaaaaggagccatcagggtttctaggatcatctcctctatccagatgacagccctctcttctctttttggacatgtttttcattttggtttggaaaggataatgtcttctgtgttctgagaagttactttttgcatttctctcctctctttctcatttattttatgtaaagccttattagctcccacaactttgtttgctctcttacttgataatggagaacataagagctaaagtcaagtggaggaaacaagttggtggtttctacatcctgcttcttataggacccggaagaggagcacctcttctatagcctgagctatctcaacagtgttctctatggctcatgctggtgactcagatttcttgtttagtttttaagttttactccccactcctgacaaacttttaatatttttaaaagcggttaaacaacgaggtactattatacacctataaggatggctaaaatccaaaaataactgacaataccatttgctgacaaggatcaacggaactttgtggaacaacaggagtctcattcattgctggtgtgaatttaaaacggttacagccactttggaagacagtttggcagtttcttagagttaaacatagcctcatcataggacccagcaatcatgttcgtaagtatttacttaaatgagttgagaacttatgtctacacaaaaatcagcatgagaattttatagcagttttatttacaactaccaaaaactagaagtaaactttagtaggtgaatggctaaataaactgtggcacatccacacaatggaatgagctgtcaaaccacaggaagacatagatgaatcttaaatgcatgttgctaagtgaaaaaagccagtcttaaaaggctacataaggtataattccatttaagtaatatcctggaaaaggcaaaactcttatggagatggcaaatagaccagtggtttcagaaactcttggtgaaaggaattgaataggtcaaccactagggattttttaaagggtggtaaaactatctttttatgatattgtgataatactagatacatgacactatgcacttgtcaaagcccatagaacttcatggcatagagaaacttaattatacaaaatttaaaaaatatttagaaggttggaggattccaggatgaaatgtaaaatatggcaaaataatctaactgtattacaaatgcatgaaataagcgtactgaaggggatgtgagagaaaatgcttacgtaagtaagtttggaaatgaatcgagtctgtaagattaaaggcaaaaagagctctgtataagcactcaaacttataaagttatttctatgtgggtatggcttaacaattatggaagtactctacaggagactggaattgaacaatgaaataaacgaatggctgatggcagaagccaggttcttcattgtaggagggagaggaaacaagcaagggggagaaggttagaattatctatgtgctactgggttgggattggagacatcagtatcaactcatatttagcttaatatagatacagatagttacaaagagaaggatttgtagatatatgtgtatagacatgggttaatttacacacatatatgttatttctctgtcagctgagcctagaagcaataacacctttgcaacaaggagcatgtccaggtcttggtttctaatacattctccaataaaagaaccaagctccttggagacatggactctaggatggagcaggaaatatacaagacgaacctagagcattttgtagctcctgaaagtaagaaagtgctcaaccaaatccaataatgacagggctatgttacagggacacaggagccaactgaatgtattctccatggccagggctggaacaacttgagcaacaaaataaaatagtattgaaagtgcaaaatagatatccatgagaccataatgatacaaacaaatgattgaataaataaatcaatgggggacaatagataaatctcccgggcagaagaagttcaaataatttctgtagatattttgccatcaaagagtggagtataaatcgctgcttcttaattgtgtgctatgccttgtggcttccttccagagtataatataaaaatgtggggaggtgcagtgggggagaagggctgtaatcctagcgcttgtggaagtcgaggtgggaggatcacttgaacc

SEQ ID NO: 13803 - RNA, 2835 nt, Homo sapiens
  source 1..2835: mol_type = other RNA
gctgggattacaggcatgagccaccatgccgggccgagactctgtctgtttaaaaaaagaagaagaagaagaagtaaaagaaggcagctcagctggtacagtagaaagcctattctggaaactgccatgatggatggctaataaaatattggagatacttaacccttagccaaacagtatgtgtctgtgtggtgtgtgtgagtatgtacatgtatgatagactgtgtgtgtgtgtgtgtgtgtgtgtgtgtgtttgtgtggtgggggtatgtgtgtgaaggccccagaaggtggccctgggacaaagcgctcctaccacttgtccccagcataggacagccacacaattcagagcacaggagagcccacacctggaggctgggctgcccttgcgggtggggttagcaatagctaacatgaaaacttccagatagcaaacctcccctggccacctgactacatatttcaaacattacctgaagcaatgaaattcaagagcattcatagtcttttttaaacttctgactacgacccacattgaggttagttacatggctgccaagggggtggggacacaggataggtaacaagagttcagactcagcctgatggcacagggtgcgctttgccctgtcccagtccactgtgtttgtggtggtgacccactaaattgattttgtgacccacttgtgggttctactgcagcttggacccgcagtctccgtgcacatggaaaatcattccctccacggaagtgggtggacctccccgcagcaggccccggcctcagtgaggatcaccaagtgccaccaggcccccacaaccccgctcaggaggaggaagcaggcttccctgaccatctttaaagaaaagggggcaccatgatgggcccactcaggtccaggctggcaaccacaggtccacccgtccaagacgcaaggcgaggctgggccattccctgcaagtgcgtgttggtcccttagggcttgcccaggggcgcccccgcgctctggcatctctgtaccaggaggatgagcctggcgaggtctgagagctccgggaacgcggccatcacgcggtccacctggtcacgcgggaagacgctgtagagcgcgatgcgagcccgggcgcgcgcgtccccctcgtcgtcctcggtcgcgtacactgaaagtcccccagtggcgccgtcgccccaggccggctccgcccagacggagcgcccagggaagcggtcggagcggggtggacgggcccacgggtcgtcgggtggcctgcgcggggaaagcaagtcgccgtgcaggtccctagggcggtgttcgccccgcggctggagctgcaggccgggcggaggcgggaggtcgcccggggagaactggctctccgggctagggaggctgagcgggcctggcacccggccgcccgcggacacccagtcgggcccgcccagtcggggcgtgaggctgcaggcggggaccgggagaggcggccccaggggccccaggtcgtcgctgaaggccagccgagagaagctccctcgcagggcggccaggtccggggacccccgcgccggcgggaggctgtgcgcaaatggttcccggggggccgcccgggctcctgcggagccgcccggggctctcggtggccgctgctcctcggcgcccgcgccaggccgggcccctgtcttggcgcggagctcgtcggccaccgccagttgcgcgtggtgcggcctctccgggtggtagaacttgcacttgatgccataggtgcatttcttgccataaggacaatgctgccaggatggctctgggggcttcggcttcctgctcaggaagttgctcagggagggtccatggcggcccagggggtcatcaggcggcatgaaccggtcgttgacgaaggagaacatgagcagcctctgctcgatgaaccacttccactcggggttctcgctctgcaggtcccggtagttgtcgttggagacgatgacgccgtcctgctcgtaggccaccttcacgatgtagcggtcgtcgtagcagaccaggcgcttgccgtgcaccttgcgggacggcgtgtacaccagcaccgcctgccgctccagctccgccagcacgtgctgctctctgataggggtgtcagctcttggtgggtccttcctccaggatggaacaaaaactttgatgtaggtgtgtcctctgtccctgaaccagtcaacagccagcttgattccccggcaagagaaggtttctttatttccatggctcatcgccacgttgctgccatcaatcactatgggtcgcagagaactggccagggttctgaagtcctcttccagggctgtccccgggccacgctgggcagagtccgggaccccacaggagccccgaggcactagcctgggtgcagccgggtgctccagggcacccgggcggctgcccgtgcggataagctcctgcagcacgtcgttgaccagggcgccctcgcccagcttgcccaacacccggagcacatcctcccggtcatagcccagcttctggaagaattccatcttgctggggtgctccatgctgtgcccagcggccactggcgcaggtcctgccccaggcttcctcctctcagagccctgcagacatgagcagcagggtgtgtccctccggtcttcacaatgaatgctggcccagtcgccagcagccttcacgccaatgttctcccgtcagtgaggccaggcccccaggtgccactggagtcagaggagggcagctggcgtgcgccaagcagccactaggagccacttcatgccaatgctccacttcctgcacgccacagtcacgttcagct

SEQ ID NO: 13804 - RNA, 2622 nt, Homo sapiens
  source 1..2622: mol_type = other RNA
gctgggattacaggcatgagccaccatgcctagccttattttatttactctttatgtaatttcaaatgttcctaacatactgaaatgataaaacgttttagatgatgggtattctaattaccctggtctgatcactatatactatagtgatcattgaaatgtcactctgtaccccataaatatgtgcaattattatgtcaattaagaaaaatgaaaagaaaaaaagtgttttaaagctgaaaactttatgaaagattacaaaaaaattgggctatgtgttttagacattctgatacaataaacttggtaaattattaggcaaattaaaacacaatcattcataatttttgtttcttctctaaaaatacattcatgacaacatatgtaagaaaaatgaaggatctagtactgagaggctggaagagttatgtggaatctcagatgaaagcctgtgtgttttgcctctaactttctaggtcacctgaaccctatgtgctcttagttatgttgcatacttttttctcatgcagtttcctgttaataaataaaaacgacatggaaaaatgagcaaaacactattaagccgaaaaatgtaggacagaaaatgatttaaaacatatatgctggaatgtacatacatatgttatacaaggtaaaaaaaggttttatggaaatataccaaaatgctaattacgttgtattatagctcagggatggatttaaggacaagtttaactttctcttttaaattattttctgtcttccaaattatctacaatgaacatgaaatgcttttttaaaaaaaggggaaaacaattttattttagaatataagactgaaaggtgctacatcctaataatttaaaaaaaaaaacagtaaaaataaatctaggattttctagtacaatccccatttcaaatgttttgtcttatatccctataaatcacttttatttctgaataactattacattttagcattgaaactacaacacaaactttgtcgatcatacatgcaagtggcacaaaaatatcttgtaatgtgctatgtccacacttcaaaaaagtattttttataaaaagtaatttcagcaaaaacacattaccatgacacatgagagtcctgcaatggcaaacatatatcctagatttatttaaagtttaattctgtaaaatctgtcctatcattggactataattcaaactaacccatctattctgaaggtggaaaaaccagtcattttaaaactgcctaatttttaaagataaattttaaaattcaactgcctacttaatcttcctaatcttcactaagtggttttggcaagatggttacttaaaataatatgaaaaaatgctagatatgtataaataattacatccatcattaaattgtgagtggattaaagtctccaaatacatgactaagatattagaataaattaaaaaaaaaaaaaaaaaaaaaactcaaggcaggcagatcactcaagccaggggttcgagaccaggctgggcaacatggcaaaacccctcctctattcaaaaaaaaattttttttaaacaactatatgcttgcttagaagaaacatactataaatataaggactcggaatgatcaaaaaatagaaaatgacacaggttgagtatccctcccttatccaagatgctgaggaccagaagtgtttcaaatttcagattttggaatatttgcatatacataatgatatgatatcttggggatagaacccaagtccggatatgaaattcatctatgtttgatatataccttatacacatagaatgaaggtaatttaatacagtattttacataattttgtgcatgaaacaaagttttgactgaggtttgaccacaatctgttatatgaggtcaggcatgaaagttttccacttgtggcatcatgttgttgctcaaaaactttcgaattttggagtactttgtatcttggatttttggattacagatgttcaatctgtatctatttcatctataaagatgatggatggttgtagctttatggcaagggagaagacagcagcagccaatttctgagattctccataccacttatcggtcagtgtcgaaggctgaaggttaataaatcgacagcctgcttctttggctgtggccttggcaatcaacgttttaccacagcctggaggcccatagagaagaacaccttttggaggctgcagaagcctggaattctcaaacaaatgtttctttttgataggtaagatgactgtgtctttcagatccgtaatgacatcatctaaacctgctatatcactccaagtaacatgcatattaagagggtctacaagatgagcagcaatactcatttcatattctgagagcttcacatttttcactccaatttgcttcattagtttttctgcctgtttctgagcttctactttttgctttctggttggatcaattgcatctaccatccatttgatagtaaagtatgtcactgcaccaaatattgtcaaacggaaaattaaaccaacaacttcattccgactcaaaggacgagaaaaggcttcagcatgtaccatcttgaatgttaacccaggggcagaaacagcaagagcaagtgc

SEQ ID NO: 13805 - RNA, 1057 nt, Homo sapiens
  source 1..1057: mol_type = other RNA
gctgggattacaggcatgagccaccatgcctgccctcggagctgctaaatgaacagccagatgaagagatacacagggtgaggtctggaagggtccttgtggagttggggtgcaccatcctcccggcacatggatgtgttcgccaacccagcagctctccatgtcctgtctttcaaggatttttctggaggctttgtcacgcaggcatgatcgagctccagctctgctccccaccccagaggatggggaatggggctgaaagcactaagcttccaaccatagttaggtatttttggtgaccagtccccaaataaggagcccaccaagagtcacctcatgagaacaaaggacgctcctatcatgcagaaaattccaagggatttaggaatccttgtgtcaggaaccaaggtgaaggaccaaacgttagaacaaaagatgtgcaatcataaaaaagaacaagatcatctcttttgtaggaacacagatggatcttgaggccattatcctcagcaaacacagctgatttccagaggatggaagaagtcaggaaacttgggacaccgctgctgaggtccttgcagccccacggtccccaggctggtgactggtgggggagtatggagtccagctgaccaccagagcctgcacgcctgctgctacaggggaggaaaggatgacttctacctcctttccacattccaaattccacgtgactaccttttattggcagcaccctgctggcaagggagccttgatgtgtgcttcctgggcttccagcacctcttcatcttcctcatccaggtattttattttaatactattcagatcaaatgaaacttttaccgaaactggagacctccattagggcggaaagagtgggggattgggacctcttcttacgactgctttggacaataggtagcgattctgaccttcgtacagcaattactgtgatgcaataagccgcaactggaagagtagaggctagagggcaggcactttatggcaaactcaggtagaattcttcctcttccgtctctttccttttacgtcatcc

SEQ ID NO: 13806 - RNA, 1861 nt, Homo sapiens
  source 1..1861: mol_type = other RNA
gctgggattacaggcatgagccaccatgcctggacatatataggaatttctaataaaatttcaagcatatgcaaaagtagaaagaaaaatacagtgcatctcaaggaacaaataatccagtttccatgatcaggcagactaaccttgtttcatacactaacctccactctaccctcctaagggaaaccccagtcatcctcttaaccatacctttcaatgtgcatctctaagacacaaggctggtgtccaaattgggaagaatgaatttaatgatccttctttgtcaccccgagcactgcccatgaggaacctggacacgaggggtgtgcttgacaaggacagacacgtggaaatgaagacgctctgcgtgggtttgatccgcaagagatgcccccacagcaagccaaatgcaatcattaacagtgtcatgtaacacggcccttgtaaggaaatcttccacacctttcttagcttttctggagaaaattctaagccaacaagaaaaagagtaaaaaacaccccaaattctcctaatgtctccacttgcacaatagacttaatactatttagtcctgaaggtcccagaagtacaccacaaataatataaccaaacattgtaggcaatcctatggctgtacatagccagccacaaggcaaggacagcattcctatggtaacaatgtcctttataaagtggtgatctgcacgtgggatggttgaatctctgggcttggtcaaaatatactggttgttctgggagtcaatcagcatgctaagacccaagtcatcctccacttctcgttttgttatattttgcttagaattggcctcttcttcctccaccctcagaactgcctcaaaattgacccccttgactgatttattgtcgtcaaaagcatgttcctctatctcttcctccagacgatccgctgcctttcttacatcttcaagaatctcgtcaagcatggataaactttggttttgatgttgcatatttttaagggcttcaacttgatgtttttctgctgccagaagttccatatattctgtttcttcctttattgcagcctctctcagggcctccaggcgctgccggctgctctccttcatgttcacgacatctttgtaatccccctgcagggctctctgcagtccgtagacagcttggaaaacggaattttcactttcattcagctctttctggaaaatttcaaacgtgtgcacctgaaacagtttctcttcatccgacaggcccacgtctttctccactgctccaattgcagttttcagtttgttcagaactgcattcttctggcggagaagccctgagagcttcctgcagctgtcccggacccactgccggctctgcatggcagccacccctcgcccgcggtgcagtttgatcacacgctgcgccacctcctcgtgctccacagcctgcaccgcccagggaaggacgggaaacagcacccagaagaagcttcttcccaacaccttcatgatccaggtccggagggcagggcacagcaatccacgggtctctgccccactgagcttgcatgtcagacacacattttcagcgggacgcagggatccgcgcccgcccgtccggcccgagcatcaccgttccgcggcctgggccgggctctgaggcgccaggacccgaggggcggagggggacgctgtctcccgcctcggagcgcagcgccggagggcttccttgcatcccttcccaggcgggaccagggaggccgggaggccgggagtccgggagggagcggccgccgccctgcccagcaccgcccccgctcagccaagccgacccggactcccgcccagccgcagtcactgccccctttaa

SEQ ID NO: 13807 - RNA, 1321 nt, Homo sapiens
  source 1..1321: mol_type = other RNA
gctgggattacaggcatgagccaccatgcctggccaaaatcatgtgacctttatattcagccctctggccaatggttaaaagcctgggcttcagagagatggagaatgagggtggggggcagggcatgatcctcccattgtcaaatttgaatgtgagaaatacagaaatgtcaaaaatctcttattccccttaaatcaaagtaaatcctatcctgagatctctcctggtatgttgagaaattcaaatttggtcattattggaactccctacccctaaattcatgactgtgtgagagaaacttagggtttcatgaagactcgaatatttaaaaaaggcttccaaaatgtatgtctgtgctggttatccatgatatgaactttttttttctaagtagaaagtcctttgcataattgcatcttcaccattgtgtgtcatagttgaaatgagttccttcttgagacgagaagttccccacacccaggcgtcatgaccttggtgtgactcaagatcattcatctctgagatccaccaacttgccagggagttgaacagaagttagccttgttctctttccagtcttggagaagctcttcctttctcttgttggccaattgtgtcttcctttccaacatctttcctccattctttttcttctgggaagatctcctgccaatagcctcagcctcccaagtagctgggactacaggtgcacaccactgtgcctggttagttttgtttattttttgtagagacaaggtctcgctctgttgcccagtaaaatcaggtctttaatacaaatgttctgactcccatgcagaattctttcctgttggcacgcaaactcaacactgcagtagaagcgtgggctttacggttatcacgacgtgccaataaatcctgcgttcttcatgttcaatgctggaaccttggacataattcctcaagtcttggtatgtttaactggacctcctggtgacaccaagaaggagtctaatttcaccaccaccaggttttttgttcacttgttcagcaaatatttagggagcatacaatgattaaagagtaaacatggttcctgctgtcttggagatgactttgctccagtttatgggtgaggaaactgaggcccagagaaggtcaatgacttggccttgttcatccagatggcgattgaaggggaaggaattgagactttgctgggcttggctccaaaacaaagactgcttccaggccattatgctgtagatctctggtacaggatgatctatagggcagacctttccttgtgggctgggatcttgctcatggcagcagttgctt

SEQ ID NO: 13808 - RNA, 2677 nt, Homo sapiens
  source 1..2677: mol_type = other RNA
gctgggattacaggcatgagccaccatgcctggccaacaccaacctttagttacttgctgaatacacaggattaaggaggaagagaaagtatcaaggatgactcccaggttcctagcttggtggtcccagtaattgagagagagaatgcagcaggaagagcagctctagggggaacaggatgagtatctccacatgatgggttggaggtacctgtgagtcacatccaggtggatgtgtcctgtgggcagtgggacgcgagtctgaagctcaggcaagaggctagagttacatctttggagtcatcagcctaatggaggactgtggcatccaggtgccaaaagctagggaaacggctctggagagagaggggctttcttaattgacctgtatgctttgaagctctatagagacacaatcttatcccttcaggcctgtattttcttgggccactaagatgtggttacatattttctctcacatctcctagaacgtttgcaaaacaattcccagtcctatgatcatttctcccttcttctgagaactaattatatatggcacttaatatctattcacatgtagcactcatggtgaggtgttttttttgtttgtttgtttttgtttttttttttttgagacagagtcttactctgttgcccaagctggagtacaatggcactatctcggctcactgcaaactccgcctctagggttcaagcgattctcctgtctcagcctcctgaaaggctgcgattacaggtgcccgccaccacaccccgctaatatttagtagagacagggtttcaccatgttggtcaggctggttttgaactcctaacctcagggtgatccgcccaccttggcctcccaaagtgctgggattacaaggtgtgagccactgctcctggccttatggtgaagtcttgtatgtagaagatcaataaatgttcatcttcattgcttatattcatccggttctctgtatacaaaatgatcttctttttgcaggcatttttttgcttctcaagttttaacttcttacacattttaagactacttcaagattaatttgagtgtaaatgagcagtacttgttaggtaagtgtcttccattcaccgtcaagactgaatcattcttttcattatcaccacatattgcttattgtggaatttggaaacatccatttctcttcttcaggaagatcgtggagtttctccagtcaaggtcccactagagtgagttagggttgcagtaacctggagtgagcaatccctgattccaggtggtgatgtgggttgagtttcacattttactttatttgaagaatatgtgcaaaagactcactaaaaataagaacaaactaggctttgttgcagctgagtggtctggcaaatttctgtatagaggaatcattgggcatgaaggatttgatactgggatagaatccaattgcccttggaatggaagtagaatatcctttttaagagcactgaagttctgggatttctccggaataatcacctttgtgatgtgtggatcatgtccagggactgtaacatttattatataagacccaggcaagagaaggagataatactctccatatttgttggttctataggggcagatatgttttctgtcttggacttccacaattacattgggtaatggatttccattctgatcaaaaacttgaccctttacacctaggtgcacctgctttatatattcaattaatgaggctttgttattattccaaaaggatggaagcttctcctcacgaggatatttacagcatgacagctccaacgtaatttcaaaacactgggcccagatgtagttgtaatcttgcattccaccttggagtggataccaagagtatccatttgtaacaccattaggaaagttcattttgtttttacactcgtctcctttcttcatgttgggatttcttgaagcataggtatgtgcaagatattgaaaaacatcatcatcaggcgttaagcttcgggagtataatgccccagttgcttgaacaccattatcaaatgggtaactggccacgagggcaccaccatggaggtttgcagagaggacaaacgtctctgttttcagccacttcatgactgccacagtttcaggctgccttgagacattattatattcaaaagcatcggggaaatttcgattcaagtcatactggttataattttcccttccgatgctgtaataacagtcaggctttttgacggcttcaaatccatctgggttcatggaaggcatgatgtgtatccgggtactattgatcagatttgtgatttcagggtctttgccatcactggttacgagatagtcaatcagatggagcagcagctcccgcccaacagtctcatctccatgcatatttgccacgtatttgaactctggaatcccaattctgtgttcctttggaaaccgccccacaacaagaacccacaggtttctacctttcacagatttcccaatactgtgtaagtgagtgacagaactgtagttttgggcaacagtcttcaaaaacgcttccatcccttcctggcggtggtagttgaaatccagcgcagctaccaaaggcagcaacagccctagccagaggcacgggaagtccatgttcaggtcccaggcgcgcacctctacccaccc

SEQ ID NO: 13809 - RNA, 2948 nt, Homo sapiens
  source 1..2948: mol_type = other RNA
gctgggattacaggcatgagccaccatgcctggccaacaccaacctttagttacttgctgaatacacaggattaaggaggaagagaaagtatcaaggatgactcccaggttcctagcttggtggtcccagtaattgagagagagaatgcagcaggaagagcagctctagggggaacaggatgagtatctccacatgatgggttggaggtacctgtgagtcacatccaggtggatgtgtcctgtgggcagtgggacgcgagtctgaagctcaggcaagaggctagagttacatctttggagtcatcagcctaatggaggactgtggcatccaggtgccaaaagctagggaaacggctctggagagagaggggctttcttaattgacctgtatgctttgaagctctatagagacacaatcttatcccttcaggcctgtattttcttgggccactaagatgtggttacatattttctctcacatctcctagaacgtttgcaaaacaattcccagtcctatgatcatttctcccttcttctgagaactaattatatatggcacttaatatctattcacatgtagcactcatggtgaggtgttttttttgtttgtttgtttttgtttttttttttttgagacagagtcttactctgttgcccaagctggagtacaatggcactatctcggctcactgcaaactccgcctctagggttcaagcgattctcctgtctcagcctcctgaaaggctgcgattacaggtgcccgccaccacaccccgctaatatttagtagagacagggtttcaccatgttggtcaggctggttttgaactcctaacctcagggtgatccgcccaccttggcctcccaaagtgctgggattacaaggtgtgagccactgctcctggccttatggtgaagtcttgtatgtagaagatcaataaatgttcatcttcattgcttatattcatccggttctctgtatacaaaatgatcttctttttgcaggcatttttttgcttctcaagttttaacttcttacacattttaagactacttcaagattaatttgagtgtaaatgagcagtacttgttaggtaagtgtcttccattcaccgtcaagactgaatcattcttttcattatcaccacatattgcttattgtggaatttggaaacatccatttctcttcttcaggaagatcgtggagtttctccagtcaaggtcccactagagtgagttagggttgcagtaacctggagtgagcaatccctgattccaggtggtgatgtgggttgagtttcacattttactttatttgaagaatatgtgcaaaagactcactaaaaataagaacaaactaggctttgttgcagctgagtggtctggcaaatttctgtatagaggaatcattgggcatgaaggatttgatactgggatagaatccaattgcccttggaatggaagtagaatatcctttttaagagcactgaagttctgggatttctccggaataatcacctttgtgatgtgtggatcatgtccagggactgtaacatttattatataagacccaggcaagagaaggagataatactctccatatttgttggttctataggggcagatatgttttctgtcttggacttccacaattacattgggtaatggatttccattctgatcaaaaacttgaccctttacacctaggtgcacctgctttatatattcaattaatgaggctttgttattattccaaaaggatggaagcttctcctcacgaggatatttacagcatgacagctccaacgtaatttcaaaacactgggcccagatgtagttgtaatcttgcattccaccttggagtggataccaagagtatccatttgtaacaccattaggaaagttcattttgtttttacactcgtctcctttcttcatgttgggatttcttgaagcataggtatgtgcaagatattgaaaaacatcatcatcaggcgttaagcttcgggagtataatgccccagttgcttgaacaccattatcaaatgggtaactggccacgagggcaccaccatggaggtttgcagagaggacaaacgtctctgttttcagccacttcatgactgccacagtttcaggctgccttgagacattattatattcaaaagcatcggggaaatttcgattcaagtcatactggttataattttcccttccgatgctgtaataacagtcaggctttttgacggcttcaaatccatctgggttcatggaaggcatgatgtgtatccgggtactattgatcagatttgtgatttcagggtctttgccatcactggttacgagatagtcaatcagatggagcagcagctcccgcccaacagtctcatctccatgcatatttgccacgtatttgaactctggaatcccaattctgtgttcctttggaaaccgccccacaacaagaacccacaggtttctacctttcacagatttcccaatactgtgtaagtgagtgacagaactgtagttttgggcaacagtcttcaaaaacgcttccatcccttcctggcggtggtagttgaaatccagcgcagctaccaaaggcagcaacagccctagccagaggcacgggaagtccatgttcttgtttgattgtaggtcataagacccccattccagaaagggtcctgtcccatacgcagaaggaagaaatgctgctcagagaggccaagaagaatctagacagacaggccttgctgggtttcctcactccatctgttaaagttacatcatacccttttgtccagtcatatttctaaacagctctacatactttttgaacctaagcataaaaatgtgcactttcctctgtcttcattctgaaggttcccatgtacacattaaatgcatttgtatgttatttctcctactagtctgccttttg

SEQ ID NO: 13810 - RNA, 2687 nt, Homo sapiens
  source 1..2687: mol_type = other RNA
gctgggattacaggcatgagccaccatgcctggccaacaccaacctttagttacttgctgaatacacaggattaaggaggaagagaaagtatcaaggatgactcccaggttcctagcttggtggtcccagtaattgagagagagaatgcagcaggaagagcagctctagggggaacaggatgagtatctccacatgatgggttggaggtacctgtgagtcacatccaggtggatgtgtcctgtgggcagtgggacgcgagtctgaagctcaggcaagaggctagagttacatctttggagtcatcagcctaatggaggactgtggcatccaggtgccaaaagctagggaaacggctctggagagagaggggctttcttaattgacctgtatgctttgaagctctatagagacacaatcttatcccttcaggcctgtattttcttgggccactaagatgtggttacatattttctctcacatctcctagaacgtttgcaaaacaattcccagtcctatgatcatttctcccttcttctgagaactaattatatatggcacttaatatctattcacatgtagcactcatggtgaggtgttttttttgtttgtttgtttttgtttttttttttttgagacagagtcttactctgttgcccaagctggagtacaatggcactatctcggctcactgcaaactccgcctctagggttcaagcgattctcctgtctcagcctcctgaaaggctgcgattacaggtgcccgccaccacaccccgctaatatttagtagagacagggtttcaccatgttggtcaggctggttttgaactcctgacctcagggtgatccgcccaccttggcctcccaaagtgctgggattacaaggtgtgagccactgctcctggccttatggtgaagtcttgtatgtagaagatcaataaatgttcatcttcattgcttatattcatccggttctctgtatacaaaatgatcttctttttgcaggcatttttttgcttctcaagttttaacttcttacacattttaagactacttcaagattaatttgagtgtaaatgagcagtacttgttaggtaagtgtcttccattcaccgtcaagactgaatcattcttttcattatcaccacatattgcttattgtggaatttggaaacatccatttctcttcttcaggaagatcgtggagtttctccagtcaaggtcccactagagtgagttagggttgcagtaacctggagtgagcaatccctgattccaggtggtgatgtgggttgagtttcacattttactttatttgaagaatatgtgcaaaagactcactaaaaataagaacaaactaggctttgttgcagctgagtggtctggcaaatttctgtatagaggaatcattgggcatgaaggatttgatactgggatagaatccaattgcccttggaatggaagtagaatatcctttttaagagcactgaagttctgggatttctccggaataatcacctttgtgatgtgtggatcatgtccagggactgtaacatttattatataagacccaggcaagagaaggagataatactctccatatttgttggttctataggggcagatatgttttctgtcttggacttccacaattacattgggtaatggatttccattctgatcaaaaacttgaccctttacacctaggtgcacctgctttatatattcaattaatgaggctttgttattattccaaaaggatggaagcttctcctcacgaggatatttacagcatgacagctccaacgtaatttcaaaacactgggcccagatgtagttgtaatcttgcattccaccttggagtggataccaagagtatccatttgtaacaccattaggaaagttcattttgtttttacactcgtctcctttcttcatgttgggatttcttgaagcataggtatgtgcaagatattgaaaaacatcatcatcaggcgttaagcttcgggagtataatgccccagttgcttgaacaccattatcaaatgggtaactggccacgagggcaccaccatggaggtttgcagagaggacaaacgtctctgttttcagccacttcatgactgccacagtttcaggctgccttgagacattattatattcaaaagcatcggggaaatttcgattcaagtcatactggttataattttcccttccgatgctgtaataacagtcaggctttttgacggcttcaaatccatctgggttcatggaaggcatgatgtgtatccgggtactattgatcagatttgtgatttcagggtctttgccatcactggttacgagatagtcaatcagatggagcagcagctcccgcccaacagtctcatctccatgcatatttgccacgtatttgaactctggaatcccaattctgtgttcctttggaaaccgccccacaacaagaacccacaggtttctacctttcacagatttcccaatactgtgtaagtgagtgacagaactgtagttttgggcaacagtcttcaaaaacgcttccatcccttcctggcggtggtagttgaaatccagcgcagctaccaaaggcagcaacagccctagccagaggcacgggaagtccatgttctctacccacccgcggccgcccggcggggccgggtgttat

SEQ ID NO: 13811 - RNA, 2413 nt, Homo sapiens
  source 1..2413: mol_type = other RNA
gctgggattacaggcatgagccaccatgcctggccaagagcttgatttttaacattagctcaaggttaatgcccccaactctcagcaaaagcatgacgggtgcccgcgtccgtctgggagtacttttcaccgttttactaaggcttcattgcccgcagccatcctgacctccacactctgaaagtgacaagccctgaagtctccagtcggggcaggtgcttgagctctgacgcccgggctgcctggcgcagagaccacgtgcttggggaggaaggctgtgtccactgggggattcctttcctcacatacaggatccagtgatcagcactgctctggaaggagggtcagggtggtgagcgttcagtccctccggccctctgagccccagcctaggccgccctctgcttgcgctcttccttgacagactcctccagctgggacagggcctcctcgtaccgaggaaccagcggctgcagcagcttgctggagagctcgtgccgctgcaactcaggtgccccagcttcagttagcattcggaggaatctcctctcctgcactttcaggagcagtgtgaaggcctgtccagttttcccagcgcgagctgtcctcccaacccggtgcacgtaggttctcaggtactggggggcgtcgtagttcaccaccagctccacaccctgcacgtcgatgcctcgcgcggtggcgtccgtgctgatgagcagctggatcttcccctgttcaaactgcttcaggatcatcctcctctggccaggcccgtagcgcgaggagaactcagccacgtccacacccccaaaagcttgcaccagcaggaagagcctgtgggagttctctcgggagttagtgaagcagagaaccctcgagaagcccatctccaggaccaggtgcaggacgaccagcggcttagagctgaggctgcagggcacgtagtggtgcgtgagcccaacaggaaaggcatacttccccgaatccccgtccccatctgtatcttccaggcccctgtgtgctagccctgtggagaaaagccggggctggtggaggcccagctgctgcagcttttcagggttctgggtcagagtagctgagaagagcagcttctgcaggggcatctggggacagcaggtgctggcggctgtcacagcctgggcctgccttcgctggagcagggcacaggggtccgcggggtcctcgctctggaaggcggccgccaccacccgcggcagccaggactgatgcatgctgtcaatcatccggtcagcctcgtcgataatcaggaagcggagctgctggaggctgaatcctggggtctggtcgatgtggtccaccaggcggccgggggtggctaccacgatgtcagccaagcagcggtacccatcagctgttttctggacgaggctctcctgctccttggccagagacttctgtcccgtaaccagggagactctcagaggtgtggcatctgtgtagatgttgaaaactttgctcacctgctgggccagctccttggtgggcagcacaaccagggcacggatgtggcagaccactctcgaaagcagggcctgcaccacagggatgacgaaggccagtgtcttcccactgcctgttggggcagaaacacagaggtcgctaggccggtagccacctctgcccaccagaaacccacaggctgcgctctccaggagggcaggaatcacagctgcctggactggaaagtaggacgagatgccgtgtgcccgcagctgcttctgcaggtcaggatggacgtcagggatgtcctcgataggaaccaggtcttcggtgacattccttctgacacagttaggctcagccagccaccttggcaggaaaggctggaccttcggcgccttcctcttcccgaacccccccagcaccaggccggggaccaggggtccggccgcctcctccagggccggtccatctggggccgcctcggcgctggcgctggtgctgcgctcccccggcgcctcctcgctgctccctgcgctgggctcccctggcgcctcctcgctgctccctgcgctgggctcccctggcgcctcctcgttgctttctgcgcccgcgtcctcgccgtccgccttccgtcgctttccctgcggcgcctccgggctccccggctccgcgtcgttcacccgccgccgccgccggggccgccgtcgcctcctggtcgccggctcggtcgatgcagccgcctcggtctgcgcgggctcccgctgctgctgccgttcgcgggcccggctctgcagccgctcgagcagcgcgcgggccctgccgtgcgccccggcctccgcgccctccggccccgccgcagctgccgcatcggggcccgggtaccgcgcgacgtagaacagcgccatggccagccgcacgcctgggactc

SEQ ID NO: 13812 - RNA, 4424 nt, Homo sapiens
  source 1..4424: mol_type = other RNA
gctgggattacaggcatgagccaccatgcctggccaagattcatggaatttttgaactccttgtcttaactactctgccagctcttgttgaacaaagaccaatccgctcttcatgatttgctcctcatgtcttcttataattctaatgtgtctacatccttggataccatataataggaaaattcttttaaacaactaaaacagacataatcacaattccaacttaatgtaatccaatacaacttcatacaaatagcagttaaatcacacgtagtaaaatttcgtacaacatttttttaaagtttcaaattcaaatgttccaaatgtttaattattttgtcttaaggtacatttgcaaagaattctaactgctgctattacctttgtccttgctgaaggaaaacattaggagaatgagctgtttttaagctaaacgtgtctccacttgatgaatggcgtgaaggagcttttccacccaagagtgatgtttctgcttcttttatttccattgcccttttgtataattcagcagctttttcaaaatctcctccttcatagctaagcacagctaaatttttcagtgtttctccaactcgaggatgcatccgacccaggctatcttcataaatctttaatgctctttcatataatggcaaagcttcaacgtgttttttcatttggctataaagaacagctaagttcaccaaggcagtagctacactagggtgctttgggccaaaagatttctgtcgaatttcaacagccaattcatacaaaggtacagctttgtcaagtttccccattttcttatacaagatggcaagatgcttcaccgtatatgccaaagaagggtgatcaggagctaatgcacgtctccgaatatctaaagctctttcataaagttcttctgctttatcatactgtttcttttcattgcatagagctgccagattattcaaagactgagcacagtcagggtgatctggtcctagaactcgctccctcatttctaaggaacgcttcagaaactggtcagctgtttccaggttattttgaagatagtagagaacacccagttcattgagggtccgagcattatcaggtgtgtccttacctaatgtaagctcttctaactgtaaagcccgtctacgtaaaagggcaaatccgtacaagttgccttttttctttatagctttctgatgaattttaaaggattttttcctaaaatgttcagcttgttcatatttattttgtttctggtacaaagttgcaagtgcttcaagttcacgagcagtatatggatggtccgcaccataagcattttctgagatttccaacgcctgtttatacagttgttctgcattgccaaacttcttccactgcacgtatacacttgctagttggtggagggactgggctactcttgggtgatcgggatctaaagctgtttctcgaatctctaaagacctctgcaaaggtactatggcctgactgagaaggcctagatccttgagaaatcgccccaaggtttcataaagatcagctaagcaactcatgttgtcctcgccttcgcagtttttctcatactgcttcaatgaatcgaagtattctgttgccattgcacttttgtctttgccaacaaactgccaataactcagcaactcagcaaagtgtccccttttataaaggttttgagacacaaagagattaagaaggcaatcatgcagcttctgtttacttccctgctgctgaaaaagccacgggagttcatctgcacttctccaagtcactctgtcctgacttagctgcaaggtgaaatagttgattagcttttgcctgtatgaagaagtaacagtggggccttccaggtactccaatctcactgtttcccaagcctgcagatgttgaaacctaagcaagccacatccataagtcaacaaacacattttgtataaactgtgaataagggaggtcaagaaagtccaggacatctcaggatagagttccatcagttctgattcactcacaccattgtgactaacattgacaaggcagaggatctgcttcattagctctttatccacatcatttgccatggactcccggatagagtgcagaacaagtctatataatgaaagagtatcttgacactggaaacactgatgaaggattttatctaaattgcctgctctcccagcacgcgcgatcattttgccgaaaagggtgacataaagggcattgcaggttgtagcagaacgacagtgtcgttctagcttcttctcctgctctttactcaatttaatgtctacagagtggcattctgcaattataatagattttgcatcttttggacttaagggatcaagatgaagtgtaggccacaacctccatgctggagggcatgtttctacattcacagaaacaattactcttacattcactggcagtggatctatcagccatttcatgtgtttttcaacttgctgaacttgatctatagaatcaataacgatgatgatgctgccttgatgacgagcagagagtttttccagccaacgtggaaattcttccagaagcttagcaggatccagtgtcagagcagagactgaccaagagtgctgcatcaactttagagttagtcgtttaataatcaaggaggactctgagctggttgacatgggccttcccacaaaatgggaaagaatcagtgtgttgggggaattcttctgttgtaattgaatccactttgataaaagaagagacttcccagaacctggtcctccagacacgagaagaggtggaatcggggctggtgctgccactagatcattaaggcgttggtaatatttctcaaatcccaactcatgggctgaattagaagcctgctgaaaagtttccatttgctcttgttcatcatgtatgtcccacagaacatcaccaaaatcatcttcttctggaatggaatcctcactgcccaaatccttagtctccaagtctgtgttctcaaaacccagtatgtcctgtttaataatcttttctacacaaatataagttttatatactccttctgcaggatctcctgagtgatcaatgatcttggctttgctggtcttgtttagattagaaacttgatcaatcaattgctggacagagtcagaactgacttttccatcttccaaacgatgaaagattaatcgaggttttccttcagggtttttcagaaaagcttcttcacagtcttccaataaaaggcttggtaatgttaagtgaataaataaaataactaaagaacttttctcaatttcccattttcttacagtgaggtattgattttcaacatctattggaaaataaacagcatggaaaaaatatcccattgtctcgcacattctcttaagtttaggtgaatagtccttaaggaaaagatccatctcaggctgggtttcatctgtataaatgaggtaacatctgacagtgttactccacagagaatgtgaaaacagaggagtaacttgtaataaactagctacagcaatatcccagtcatctctattaacatttgcaaagggtccttccacatctatagaactatgggcaaactcagggcctctgaaggactgctgaagctggatcatgcttcctatggaaggttcacttcccaaggctccgccagtccaatattcacattgggttccagcagcagtgacatctgtacagttgtcatctgaatcagactccccaggatcaaatacttggataccctgagcctgtagcctctgaagtttgctctccaactccctcttggccctcagtaagtcctgaatttcattttctttggtctccctaaaaatcttgaattgccttttaactttatctctgtcatgttcaaatgttgctgctctctccattgcttggtatttcgcttctaaagcactttctttttctcgaagtatcttctgatacgttttttgaagtgcctgcagttcggcccgcagccgcttgttctccgtgtccagcttggcctcgcggcggcccatggacaacaactcctggttcttgctgacgcgaaagatctcgtactccttcctgagccgctcgtactcggccgccgcgtactccagctctggcaccgacgagccagtggacttgaagctggcccccagcagcccgcccgcgcccaccccgcggggcagcgacccgggcccggcccctgctgccgcccccgcgcctcggcggaacgagttgcgcagcaggcgggccttgggcttcacctccaccgggatctcgcaggcctcgccgccgcccgccccgtacgtgtcctcgatcacttccccgcccgcggggctcacgagcgacgaggcggtccccatggcgtccgttgccgctactacctagtgagtaccagcaggactgggcagcggaac

SEQ ID NO: 13813 - RNA, 3983 nt, Homo sapiens
  source 1..3983: mol_type = other RNA
gctgggattacaggcatgagccaccatgcctggccaattctttctacttataaaaaattcttatgttcttggtggataaactggttgcataataaaattattttagttcaatggatagattcctgccagattcacccagttgccaattatctgaactgaaacaaataaaaatatcaagtaaatttttatatcaccctccaaaagcttgggaattatattctgccacttaaggctttactggacttactgtccataaaattttctaattacaaagtggaagtctattcaagagtgtttatacgtagaaaagttaggaagacagaaacttgaaaaagactgtcttcagaaaaacctctctgtttccaataggaatataccatggtcataattttatgctcacatgtcacacaaagataggctgttactggagagttattttgtacagttggtatttttaattctccattttttgttcacaaatgtagtcttcattttaatgaagaagagaagtctgtgtttcttccatgttgaactcctctgtccacttctgcaggtcttgtgcattatgcatcgtccataactttgcaaaatacttgagtctctttcttttcgtatttattaatccttccagctcttttgacttgtgagctgctttcttcaaaatttctccaggaacatctgctagtttagccacatttaatccataactccttgctgcaattcctctagttatttggtaaaggaaggtgacaaaatcagggacttgttctgctgcgcctggatccagtttgctttcatcctcactgaccaagaatcccatgtggtaattccccacctggtgtgagtaatttttttctagttcacaaactggcggataatgggtgacaaacagggttaaggatttcacatctctgatgaaatactcaagtgtagcataggcaatggcaattccatcatgagtgctcgtccctcttcctagttcatccaagataaccaaggactgtgatgttgcttttctgattatttctgctgtgtcagtcagttcttccataaatgtactctgtcctttatatatattgtctgcagcacccatccttgtgaaaatgccatccacaatcccaattgtcgcttcttctgcaggaacataggagccaatctgagccatgatggtaatcaatgcaacttgttttatgtaggagctctttccacccatgtttggtccggtaattatcattactctctctgagtcctctgataaatctgtattatttgggacatattgatcctgttctcccagcaacacatcaatcacagggtgccttccattttttattacaatttttctttcttcttgtacagttggtctgcagtaatctccttgcttagcgaccttggccagggagaaaatgcagtcaacagttgctaggtgatgcactgctttacacaaggagtgataatgttcactgaatttctctagaaaatcaagccattcagcactgcagtcaaggactagctgctcccggagctgattcagatgtctgtaattttctacaataaaaggagagtgaaagcggctcacagcttttgtgcttccaacctttacccaatcagttggtatacaagatacagcagagttctttatttctatcataaactcctgtcctgatactgtcacatattgtgcagaaggattttttagtatttttcgtatttcttgcaaatgcattcggatctcgtcaataacaccttgaatttcatccttcctcttttttattaaagggaagtcagaaaggtctttaaataattcagttttatccccaactttggcagcttgttcattgagtatctttaagtaatgctccactggactgaggagttcaggaatttctaaaataacggtccggagcaagtctgactgaatgtgggaattaacagcaggtattattgcttgaaattctgactttaggtgatataaagttttgacaatcaagaagaactcttgggtagaacattttttgtgataaatgctacagagtcccctctctatgtcgggcaatttacgtagatgattttctatctgaccaaacacactagattctgaatggagaacttccgatacagcatcaagccgggcatttatttcccttaatttaaggagtggctgggtcacccacttctttaacttccgtctcccaaatgaagttttagtgtggtctaaaacccacagcaaacttcctttggttttcatatcagtctgattctgtaggatttccagattccttaatgttgttccattaattgtcataaattccattttacttgatagctgtttaaaattctcaggtttggagagcatcttttccaagttgaattctttgaggtattttatgatggcagccaaagagcaaatcacaggcttctctaagttaacaatgccagaaataatttgagaacctttgatgtcaactgtatcttttgcataaaactctgtaactgcctggaaagcatggctgtattcaaaataaatgttatccatcctttcgactcgaattctgtcatcctgcacactaacagatgtggctctgtggatgagcgcctctgtttgctcggacaaggccgaaggaagcagcagctctactggctgcaggcttgacatccgggtttctagctctgaacgagaagcagagtcctggaaactatcaaacacaacctcgcctgtggcaggctgcactcccacaatgccaataaaaatgttgcccttttttttgtccctaacattttccttattttcagagatgcacagaagatagctggtagaagtatcagtcattatctcatcaacatttacagcatcatccagcttgattaggggattcacatcttctccaataagtgtagattttgtataaagggcagtcaatttccgggaaaagagtgaacttctgttgtctccaatggcctttaatgctgcagtttcagtttgcttcacaactcccaccttatatccttttgccaccaggcggcgtacatgaacaaacagtctgtgagtaggtatacttgctgtcataaagttgtgatctaaatggcaataaatattgagctctcgggctgcaatctctgcatcttccccaaagaatctatacttatatccacattccacacacaaaactgcatctttgtgctgctgcttcatttctatgtattgtaattctagcggcgtatagatgcttttggaccgtttgttagctgatttggaagcagttttctgtaaattttcatgacttgtatttgatgatccaaactgactgagatcaaaaagtgttgtgtccttttgattaatttgacgtttcgaatcttcagaagaaactgcattctttgcgtgtagaagactgatatcatcaaaatcagtacattttggcagaactgcaaatctctcctgcagagattctgtctggactctactttgaggaagggcagaatcgcagcagaattctttcaatttttccagagactttgaaacattcctggtcctcagacatttctttggctcagagttgccagacattcccagatcacttcctccttccttttgttggactttctttactttctttttaacaggcccatcattttccaatggtctcttctttcttctgtcaatttctgtagctatgtgcggcggcagctggggcgggaaggcgggagctgggggcgctgggggcgctgcggccgctgcggccgctgcagccgctgcagcgccagggtccacctggtcggctgcacctgtggaggaggaggtggatttcaggcttcccgtagactggaagaatcggctcaaaaccgcttgcctcgcaggggctgagctggaggcagcgaggccgcccgacgcaggcttccggcgagacatggcagggcaaggatggcagcccggcggcagggcctggcgaggagcgcgagcccgcggccgcagttcccaggcgtct

SEQ ID NO: 13814 - RNA, 1843 nt, Homo sapiens
  source 1..1843: mol_type = other RNA
gctgggattacaggcatgagccaccatgcctggccactggttattttttactgttgacatacttaattacaaaataataactttaaaaggtatggttcttcaataatgacacatatatcagaaggtaataatactaaaaaaaagatctgtgaaaaaactttcaaaataaaaaaattaaatataattttaaaaaatgacgtagaaaaactggatttatcatgtgtaacatgttttgaaatatctatacattgtggaatggctcaatatagctaattaacgtgcattaccttatgtgcttttttggaaaaaccacttaaaatttactcagtgactttcaaaatacattgttgttaattacagtcaccaagctgtacaacagatctcttgaactcagttgccttgtctaactgaaattttgtaaattttgaccaatatctcctcaatcctccactgccccaccagcccttgataaccaccattctattctctccttctatgagttcaacttaagattccacagtgagattatgcagcatttgtctttctaagcctggcttattttacttaacatgtcctccaggttgtcacagatgaaaggatttccttgtttttaagcattaaatactgttccatcaataccatttttaatatatttaaattatatccattttggaagtagtaacagcatgctttgatggtggctcagtagaagacattgtatcagaaatccacaaattaagcaactgtttcttatgaagtgcatcattttcctggttggcctgttcatccagtgactttcttatacaattctttaattcttcgattccttctccagtaactgcagatatggggatgatatgttggaactctacagtcctctctggaatcatgtttttttcaaataaatgcagaaaatctttaggattctggagctggctcatcaattcatggaacttatcttgggcatctggcaagtccattttattaactgccaagagtgcaggttttgtctgaagttcctctttgtacaattccaactcttttgtaagcagtattatggtttcaaaagctgtcctgtattgagtgtgagaagaaagctgaaatccagaaatatcaacaacaaaaagtagttgtctagttctttctatatgcttgaggaatttgtggcccattcctttgttcatatgtgctccttctattaaacccggaagatcagctactgatatctgtttgaaatcactgtacattatctttccaagttcaggctttaatgttgtaaatgcgtaatctgcaattgcaggttttgcatgagaaacacaacttagcaaagaggattttccagcatttgggaatcctactaggcctacatcagctataagttttagatcaaggtgaattattcgtttctggcctttcaatggtaagaaatttgtaagtaatttaccaccaagacctccttgagctaccaaaattctgtcattttctttattgagttctcctataattttaccattttcatcagttactgaaatacccacaggcacagggatttcacagtcttttcctttggagcctttcagtgcactaattttgctgtttgctcctactccagccacaaaccgtttccgaggatacctgtctttaagttgttttaaagtcattctgttctgggctacaacccagacatcaccaccttttccaccttctccacctaaacgaggataacccattccaccggatcctcccctggtgaagagtcttagcttatcgatgaaatttccatactttctgaacaacacgcaactgcaatgcaccatggctgcaacaggccaggaaaccttct

SEQ ID NO: 13815 - RNA, 1606 nt, Homo sapiens
  source 1..1606: mol_type = other RNA
gctgggattacaggcatgagccaccatgcctggccactggttattttttactgttgacatacttaattacaaaataataactttaaaaggtatggttcttcaataatgacacatatatcagaaggtaataatactaaaaaaaagatctgtgaaaaaactttcaaaataaaaaaattaaatataattttaaaaaatgacgtagaaaaactggatttatcatgtgtaacatgttttgaaatatctatacattgtggaatggctcaatatagctaattaacgtgcattaccttatgtgcttttttggaaaaaccacttaaaatttactcagtgactttcaaaatacattgttgttaattacagtcaccaagctgtacaacagatctcttgaactcagttgccttgtctaactgaaattttgtaaattttgaccaatatctcctcaatcctccactgccccaccagcccttgataaccaccattctattctctccttctatgagttcaacttaagattccacagtgagattatgcagcatttgtctttctaagcctggcttattttacttaacatgtcctccaggttgtcacagatgaaaggatttccttgtttttaagcattaaatactgttccatcaataccatttttaatatatttaaattatatccattttggaagtagtaacagcatgctttgatggtggctcagtagaagacattgtatcagaaatccacaaattaagcaactgtttcttatgaagtgcatcattttcctggttggcctgttcatccagtgactttcttatacaattctttaattcttcgattccttctccagtaactgcagatatggggatgatatgttggaactctacagtcctctctggaatcatgtttttttcaaataaatgcagaaaatctttaggattctggagctggctcatcaattcatggaacttatcttgggcatctggcaagtccattttattaactgccaagagtgcaggttttgtctgaagttcctctttgtacaattccaactcttttgtaagcagtattatggtttcaaaagctgtcctgtattgagtgtgagaagaaagctgaaatccagaaatatcaacaacaaaaagtagttgtctagttctttctatatgcttgaggaatttgtggcccattcctttgttcatatgtgctccttctattaaacccggaagatcagctactgatatctgtttgaaatcactgtacattatctttccaagttcaggctttaatgttgtaaatgcgtaatctgcaattgcaggttttgcatgagaaacacaacttagcaaagaggattttccagcatttgggaatttgctgtttgctcctactccagccacaaaccgtttccgaggatacctgtctttaagttgttttaaagtcattctgttctgggctacaacccagacatcaccaccttttccaccttctccacctaaacgaggataacccattccaccggatcctcccctggtgaagagtcttagcttatcgatgaaatttccatactttctgaacaacacgcaactgcaatgcaccatggctgcaacaggccaggaaaccttct

SEQ ID NO: 13816 - RNA, 1896 nt, Homo sapiens
  source 1..1896: mol_type = other RNA
gctgggattacaggcatgagccaccatgcctggccagaagtcatttctttatccctggacaggaatctgaacttgaacatggacaaataatctctctttcatttagcagtgcacgttatagttctatctgtattcttagccaacaggacatggggccagtgaatttatttttacttttaggtcatagccaggccagacttaggaactggtctcttatcacaggaagtttgtaattggtgacttcctggctggggcagatgtttttttttttttttttcctccaaaagtagttgctgccctatttgctgtatgtctgcctgcattcttaattctgccactgcctggtctacttacctacgctcctgacctcccaatctgagtccttccaggcaaggctgtgtccttcgggatgtatcctgattccaacatgcttgttttcagccctctagttagctctttgttgccagagaggaaatatacccagtcgtgtggtgataaaaaccacggcaaacataacaaacaggagatcacacattttctgaaacttggcataatttgccattttggcagcctccagaagagcatcagctgaatcatgaagacaaaggaccagcgttcctactcgggccatattgttgacatatgaaaaggtaatcaagaaaatagatacaaggtggtgcaggaacataatgccaaagtcctttcttttgatatcagtgaactgagaaaacatcaaagaccaataaaacgacagctccaggatgtaatagtagtgaaggtcagttgtgagtggctgataggggtagttgtaccagcaatgcctcgtattccacaaccagggggtctttttcaggaatctgactccgtaggtaaatacataaaggtaaaatgaaaatctccacatgctctcacagaacctcgtcagcgtgcttggcttctcctgattgcgtctttgtcgaaaccagcgctgaatgcttcgaacatcccagtccagttgcttggagaggccttccaatctcttttcatcaggatgctttgtaattgcagtgaagaccttttccagaatggcattgggcggagcaatttgtggtccattggcctgaatgttgagggctatggcgcacggtttggctacaaatctctcgaagatgagccgcaccatgaagatacagaaggccaggggaaaagcgagatagaggtcctcagcctgcgggaaggtggcctcctccgtgttcttcaggtccgcccaggtgacattgtgcgggagccaaaacctctcgttccagaaccaggctaagatccctgccatcttgctttgtccactcctgtcctgcggcacccgcagcccgccaagctctccaccgcgcagggcgcccggggatgcgcgcccggctggccccgagcctgtgccgccgccgccgctgctcccgcccgccgccgccgcctcctccgcggccgctgctctcgaaggctcgcggcgagccccggttctctcctccctctggccgcgctggggaaaggggccgccttgcccgtcacatggcagctcgggccgcccgccctgattggctcgtcttcgcgtcaaacagcgaggcacacacgcggccaactcgcccacacccgcagggcagggcgcagtcgctgcgccctgggcgcaggggcaccgctccggggagtgtcgcccgcccctgctctcaccgctctttcgctttgcgcttagggcgacgacctaaagtcgaccccccaaatccgccctagccccctggctggctcgcacatgctcagaatgctggctcctgccccgctggggtttcagggctctcagtcctcttcccgtgcgcccggaggcggtgggtcagcaggtaggggctgccgccaagcttcagaaccagccct

SEQ ID NO: 13817 - RNA, 5954 nt, Homo sapiens
  source 1..5954: mol_type = other RNA
gctgggattacaggcatgagccaccatgcctggccagatcttccaaaaatacttgttatttcagtaatgctttgctgaaacatttgtagatccccactgactgaaggacacagtacaagattcttatcttccaaagtccattacgaattgaatcctgctaataaccgtgtgatgaggcttagaagcagatcttcccccagtcaagccttcagatgagaccacagatcaggccagccatttgactactactccaagacaccttgatccctctggcctcagccctcagtccctctggactcagcctttgcactcagctaagccatgccaggattcctgacccacagaaacaatgagctaacaaaagtttgttttaagccactaagttttggggtaattttgttacacagcaatagataactaatacactctcaatattgctcttttgtggtaactattgcatgttgtcatggattaatgaagtttttggtatttgttatatcaagaatgagcatagcacaccccattctgttgattttctagaaatacctgtgtgatgactgattgatcaaatgttccttgagagccttgacatagaaggtacccaagaaacatgaacagattgaggcactgtctcttagcatgaatacagtgtggtttgctgaaaactggctctgaagaagaaagctgagactcatgctggtcctatgtgttactttggacctggcatttgaatctctctgaacgtgggtcctcatccctaaatgaagggctgatcgcaatgagctataatgtccctttccactgacatttgaagattccaaggaggtcacaaagcatcaggttgagacagttgcttgaagccatggagagagcagccaaattcttagctcagtgcagggaagtgtcagatcattggtccatgtgctttcagcaacacatcccattcccaagaaagccttttgtcatttctttgacacatcaacttcagaatacatagggaccctgtacttttctgtccagatgccttgattcctgcagctcattccacctgcaatgcaccttctccctctgtcaaaacagcaaaatcttcagagctcaattccggtgctactcactgcttcctccctgccaaagtggcttctgatgctcaaagcaggaccccagctctgtcaccaccttccacgattggtaataatgcagtgatttatgtaccttgtttctcttctacattataaactccttaacaacaggaactaattaataaatatttgttgacctttataaattgaacatttcatctgatttggcccttggtggacctgggggcaatattttggggctgatgtcagaggagggttttctgaataagtaagggtcagctgctgggggtgggggaaggtatttaaacgtatttctgggtttttttttaaaatgaaaaaattaatgccttaaagtgctctaaactggtgaccaacaaatgaaaaattaatttccactaatgaaacttatcacttccttcttccactacaccatcgctaaaagccacccagatattaaaaacatccacgactcctttttatgcaaaatttcctgctgctaagtatcagctctagccatctaggtgaataatcaagtgtcatttctaataagtcagtggctcctgtcaagacttgtgaccaattagaagtcaccccaatgaggaggtggctgctggcgttgccaagcaacagccaagctgtgaggcacatttagatgctcttttagatttaaccagcggcaagtcagagtgacattataattctggcaaaggaaagccaaattataacccaggctggggtgcccatgatgaggagtgtgttttcttttaaatgcaaatgcaaaaggaacatttaaaccagaatttaaacagtccatcatgatagtgattttaattagtagatcaggtgtcggtggaacacgactgtgtctcaggataatggtctctcgctgctagataaatacccagctattccagaaaatgggcaactggtcaggcaaggccaatgtatttttggactctgaagtattgatgactacagccacacttggttataatgacgttcatttttattgttcaggaggattaagaaataaaagcaaatattaaaaatagactgctggaaatggatgcctcctagagaaggctgcttgctctaatgttattgggaagcgtgttctgccttagaagcccccatatgtgaccatctggagagtttacagtgaaaatttaaaggccaaactaaactgtgatgatgactgtaattctgaaaagacttttgcactgaaatgcatttactcataagcgggctatatcaacttaaatttttaaaaattgtagtcattctcgagtaacatgtcgtctccaagtcaggaaatgcctacagggagtaataaccacatctgcctctgcctttaagattcatacattattgactgtgccttcttgacggggaacatctggatgaaaagtgaaaaattaggcagagagccggatcagtgctgtgcgagataccagcctcccattttatctgacttttctttaactgagtccctatgcatagcaacatgattggttcatttactcttgagtgacacatatatccttaggcactcatctatgaagattcattgtctcccatatctgctcaatggggtaccatcagctcttagttatctgggtgaatgaagaaagcccatcatttatattgggctttgagaatggagaacatacaagctgccatattggattggatccatggttaatgaggtttgaagcttagtctctgctagaggcactcaaaaactgggttcttcatggaagctacctgcaaaggataattgctcaagagactcatttctctcagtagccaaccaggaagttaacaacccacgttctctccttttgaaaacctatttgagcccagaataaacaaagttaagcaggtttctttactgcaggcctttctcaagcctttcatatgctcaggtacatggtgaatcttgaagaatatagtttgtaatatttcaccaaattatttgactatggggccttttcggtcctccatatttcaaatccttttccctggtagtaattcatagcttgaaattcatcatcatataagtacagtttagatgcctttctcctaaatgtattcttttattcttgcttacactgaaggttacctgccacttttgtgctgacttatgcaatcttacaagagtctcagaaagttattcctattgatttaatatctttcaaatcagaacagcttagaggaatatacaaatatatagattccactgtgttctctctctttcagatgagttataaaatttaaaaataaatctagtgctaacctgggtccccaggggatcacattatttatacattttccgtcagagaagtactaatttagccccagttttatttcctgaaattaaacctatttattccctcatccttaataaagttttacacaatcccagggttactactcactaatagtctttggtaaagaatctagcaaaagactgtgaaaatctaaatctacagttgtgctttttaaaacgtcaattcttcgggggatggagtgaaaactctggccagttaagcagacaaaatcttccctaacaacagcaacaacaacaaaaagtcagttgtttttccaggaatgctcagccatccttttctataaatcccaataacttgtttgtcgctggctatgattccaatagtctctttttcctgacttggagatgcatgaatcacattttccctggttctctgttgctctatattatccctggtatgacataggccaaaaaaaaaaaacaattttaatttaaatacaaatatggcttcatgatatgatgctcattttaaagccattttcaagcattgttgactgaggcaacctaatatccgcataaacgaagacaacgccatccaaagcttttgaatattgaccatacttaaagacacaggtagagagggacttaggctgccaaggttctaaaggagaaagcctcagaattccaaggggaaacaaacttttatttcaagaataaactctgatgtttgataacaaaagtccaaagactacttacaaattcagaaaggactagagatgctggtatttcaaagctatttccaggaaaactgactcagatacccacagccgagtatctgtggctcagagtctctgagctatctcctaacactgtggctcatttccctctttgtgtctgtgactttttgtatgtgtatacgtatatgtgtatatatattggtgactctctaaaggaaaagccagtttgctgtatcctcttatttaattttttcttgatagaattatttccctttcatttttttagcttagtttcatcatgtatccttaggcagaataggtagaaagcttctcggttctttgattcttcatacatccattcattaattgttcctgaatgtctattatgtacctagtgtgtgcagttaaccataaagaaaataagaaaaaagcaaaaagactttgtcctcctgaagcatccatctagcagaaggggacatacaataaacaggtaaacaaaatggaatgttagctggtgatagttccacagagaaaaataaagcagtggagggtgggggttcaggggccaggtccttcgagcctggagatgtagtcggtctgaggtggtcagagaggggaccaacaggaacactcactgtgccggggctttccacgctggctctcagcagaatctttccagggaactcgtgacatgcgaattctcagttacccttagaaattctgactatatagatcttgaggtggctgaaattatgtatttttaacaagggtcctaggtgattctcatgcagcccttggtcccacaaggtttgagaaccagtgacttagagaacaaaggcagctgggagattaaagtttgaggaagcatccagaaaccaggaggttttggggaggaatataggacacttctcattttgtcccctccacccatcttccacagcccagaagcagcccccctgtcatttcctgcatcctgtctacaccatggcttagagcctcaaaccctctgctcttcatatgcaaaggggagctgcttttggaattaggaaaactctttcctctcctaataaagcttgctaacgtacagttcaaaatcaagcaactacttccttgttctggatggcacctactgtcttcctcagaggcaccttcaggagcacccactggtgccattgattccgcgggtgcgggaaaattacagggaacacgatctatggagcatgaaacagacatacattggtttcacgtttcagaaatattatctttgctgtgcactttttcgtcctcgtgtttctttccatgtgagcagcatttaacacctctggctgctccttcctctttgaaatgctttccccttccacattctgctggtttccatttcaggctgttcttcctgagtcttctttataggtttctcctccgctcctcccttaaatatggttctccccagaaccatatctaacacatatgctacacgtctctgtgttttgaagaccatctttcttccccctcccacctgagtgccatctgcacagccaacttcttcttgaagggtctccttaggggccttccagtaaacttcaactcgccaggtctaaaatccccagaggtggggaaaaagttaacttctcctgcctctgggatggaatcctttcaaacgcaaacccaagaacctaaattgaactatatggagtagaaaaaaatgcctttcaagggaatttcaaggttattgatagtgtatggtaaataatgggctctatgaaatctctctctacctcttggcttttttttttttttttttttttttgagatggagtctggagtctt

SEQ ID NO: 13818 - RNA, 4281 nt, Homo sapiens
  source 1..4281: mol_type = other RNA
gctgggattacaggcatgagccaccatgcctggccatgtatacacatcttaatacaaatattttcagagataaccattgcgtgatagctattttttttcttgaaatgataccctccttcacccttttctgtcagaactgaaagctacatagcttcttctatttcttcatgcacttgttagaagcaatatgcattaacctattttccgatgctgttgattctctaatctgttaatccatttgcagacgctattgattttcaaacttaagttatgaatacctgctataattctgtggttaataaccagctttggaaagaaaatgtgcttctatcaaagggtacaatttttctatgactaaaacatataaattcatccatgagcaattgcaagtgtccaaacatttaccctttctgaacaacattaacttcgccagggcaaaacaaagtcacacatgtaacatattccccaagttgccccactcccaccacagtgcatatgtgcacacacacacacacacacacacacacacacatccaaagcccagatttcatgtaaaaaaaatctccccttaagtaattatttttcctactgcatatttttaatctcgttgtctttgtatatgaattgtctttcctcttatattccttttacagaatttgagaaatgaaacactgaggaatgataaagattatacatgtattcaaacaatattaaagacatataggtcaaaaccttttctgatatctaaatgctatgagatcatccctgtattaagatctgagtcatgattagtcataatatacaggtcaatatgtatattctcatccaattatctttagaagtttctacattatataactcagccctacatgcctcaatgattaaaaaactttcctttatattagatggacatgtccacaaatatcctaatgcaaatagaataaaccttgtattatcagaagaacatgtctacaatgttatcttacatattaatatcttggacagatacttcttttatcttcccagttaaaaggaaaggcactaagtatgctttaagcaccttcagagatgcaaaagatctttccaaacaggtagattcttggtttgtggcttttctgtagtaatgctcaacatttactctggcggctatcataaggaggaggctaaaagttattttcgattttagtatccaaacaggccagttactattcctttgtcctgtatccttctgtgggtaaaacacaagctagaatttggtttatcttccctttctatgctggagctttttaggagaactaatgctctcagaataagtgaacccctgctcaagaaacagagttacctattaatgtgtctccttatgaaaaaggaaaaacctttgcaattgtcctactgctgtaaaggatgaaaccaaatgtctttttgttcttcatccaattagcttaaaaaattagcctagaacaaagtggtagaaatttagaaagcatatttcagcaaggactatggatttataaagaaatgtggattcagataaaatatacttcagagagaaaattaggataaacattttatgacacaagaggaactagaaaaagcacaggaatttaaggaagaacatattttaatggttgaaacctgtctttatgaggcgattatgacagcaaaaaatattataatgaataacaatgcatagtctacgctttgtaatatttcatacaataattcctttatcatttacatctcttaatgctagaaaagcattctgaagatgccaagcgtaagttgcaactgagtaaaaaaaaaaaagcaaaatttactcaatttccagaagaggtgcagaacagagaatgaaggtccttaaaatataaaccgctagtgtgctaaaatgatgtccatttgcaggatcagtgacaaaatatttaagcccataaagaaaagagttatacctgctgtatgaaggtattcatagagaaatatgagtcataagccaattatttataaatgtctttcaaaatatttggtgcacatgaaatgcagtatactgatggtcctggagactgttgcagttgaatagggcagctactgggatgatggtgtttcccccggatgaggatgacaggaatgcagggcctaggatttgttgagcatgtacactcttcttctgaattggccacccagaaaccaattattgaatcagaacaacacaaattggtttgtgcttgagccaggtctgtagaaacggaaatcaattcagttgtggaaatgatgaattttaaaagctgctgggtttttttttgtgcaaggtagagattttcataacatctcaataatccttttgaaatgtgcagttgcttagtgcaaaaaaagaaatagtgccaccatttcttcaactaaaagataaggtgtgctttgtaaaagtaaagcatatccaattttcatcctgttggtcggtattaccaagggtcatgatgtagctggcgcacaaatgtgaagaatcatttactacttattttattgttttcgatctgcatgcacaatatgaaatcataaaagcaacaaacatcaccacaccaacactgagtaagatcatttctatcaggccaaggaggtttatttttccagttacttgacttctgaacatgtttgccttctcatcaccaatggtcccagtctcattaagccaaagaataggcacaatatagttcctcttcagattctttaatacttgaattttttctgatggcttgaccaataggttgacctgcagccgttttgcaaattgtaaagtgaatccagttataggttcaatatccaagtatgtcctatgttcttcttcatttgggtttaatccatcaataggttctgaaacatcaggacttgcatacagaaaatgaggaagtgaaatgtacacaggtctcccttctttgcatttgctgatgtctagcacaccatatgatgtacaattttttgagataattttttctgtgcagaaacaatagttgtctgggttttcaactggagaggcaaaggccttggatggaagaacaaatctatacacagggattcctttcagattaacgtcggattcaaatacagcatagattgacctgcaaatatcagaagaaaagaactgcaatacctggcttttctcaacaaaaggtggaaatgaggctgcatctgtaccattaatcatgtcgcagtgactttcccaataggacagattccttttacctttatatgtgtcgattatggcaactttacttatgttatcttttccattgaaaactttataaactccatctgcagtattgttgtaaggataaaacagaccaactgtggtagtaacagggtacggaaccaaactcaaaaatggatccctatagccccataacagttctctcaaagttctgacttggaacatagaagattttgacttgttaataagtgaattgaggatcatttgaacaaattgattttgatagatatgggatgcagctgccacagccagattgagaactgtgaagttgtcagcctctgttccaactgatagtgaaggttcgaagatggcaccattgggctgcaggaaagagactgtgttgtcctcagcgtcctgggttacattttccttggctagaaaacgaactctgtacgtataaggacctctttgcttaacttgaatgttgctgctgttcatcatcacttcctgtggattttgcacatcaaagatccaaaactgtctgtaaacttctgtgcctgttttaacccaatttttaaaagcaattgtaccttcttcgaggacaacttgctttttaattgtcttctggataagcaggtctccaactggcattagaatacctccaaacacagccaggacagcaccaatgacagccccagcgatgagcccacagttccggtcacagcccatttttcttgttcaggaggtgaattagtgttaagcacctgtttcttgcaaactcctggatatgattaaagtggtttctacaagctctggttcttattcacaaatcaacagcaagacatgaattttacaggaaatgaactgatgagtcacagaaagaatcaattcgtctaatcattggaaagctatcaacttctagaagagcttgctttcggagatgtaggacctcaagactggctccagagtcttgcaggagcagatgcagaaagtaaacaggatttccacggcatagcagctgagaactcagaaatgaggcacaggctctcaacccttcatctatccttaaggttatcctgacatct

SEQ ID NO: 13819 - RNA, 4214 nt, Homo sapiens
  source 1..4214: mol_type = other RNA
gctgggattacaggcatgagccaccatgcctggccatgtatacacatcttaatacaaatattttcagagataaccattgcgtgatagctattttttttcttgaaatgataccctccttcacccttttctgtcagaactgaaagctacatagcttcttctatttcttcatgcacttgttagaagcaatatgcattaacctattttccgatgctgttgattctctaatctgttaatccatttgcagacgctattgattttcaaacttaagttatgaatacctgctataattctgtggttaataaccagctttggaaagaaaatgtgcttctatcaaagggtacaatttttctatgactaaaacatataaattcatccatgagcaattgcaagtgtccaaacatttaccctttctgaacaacattaacttcgccagggcaaaacaaagtcacacatgtaacatattccccaagttgccccactcccaccacagtgcatatgtgcacacacacacacacacacacacacacacacatccaaagcccagatttcatgtaaaaaaaatctccccttaagtaattatttttcctactgcatatttttaatctcgttgtctttgtatatgaattgtctttcctcttatattccttttacagaatttgagaaatgaaacactgaggaatgataaagattatacatgtattcaaacaatattaaagacatataggtcaaaaccttttctgatatctaaatgctatgagatcatccctgtattaagatctgagtcatgattagtcataatatacaggtcaatatgtatattctcatccaattatctttagaagtttctacattatataactcagccctacatgcctcaatgattaaaaaactttcctttatattagatggacatgtccacaaatatcctaatgcaaatagaataaaccttgtattatcagaagaacatgtctacaatgttatcttacatattaatatcttggacagatacttcttttatcttcccagttaaaaggaaaggcactaagtatgctttaagcaccttcagagatgcaaaagatctttccaaacaggtagattcttggtttgtggcttttctgtagtaatgctcaacatttactctggcggctatcataaggaggaggctaaaagttattttcgattttagtatccaaacaggccagttactattcctttgtcctgtatccttctgtgggtaaaacacaagctagaatttggtttatcttccctttctatgctggagctttttaggagaactaatgctctcagaataagtgaacccctgctcaagaaacagagttacctattaatgtgtctccttatgaaaaaggaaaaacctttgcaattgtcctactgctgtaaaggatgaaaccaaatgtctttttgttcttcatccaattagcttaaaaaattagcctagaacaaagtggtagaaatttagaaagcatatttcagcaaggactatggatttataaagaaatgtggattcagataaaatatacttcagagagaaaattaggataaacattttatgacacaagaggaactagaaaaagcacaggaatttaaggaagaacatattttaatggttgaaacctgtctttatgaggcgattatgacagcaaaaaatattataatgaataacaatgcatagtctacgctttgtaatatttcatacaataattcctttatcatttacatctcttaatgctagaaaagcattctgaagatgccaagcgtaagttgcaactgagtaaaaaaaaaaaagcaaaatttactcaatttccagaagaggtgcagaacagagaatgaaggtccttaaaatataaaccgctagtgtgctaaaatgatgtccatttgcaggatcagtgacaaaatatttaagcccataaagaaaagagttatacctgctgtatgaaggtattcatagagaaatatgagtcataagccaattatttataaatgtctttcaaaatatttggtgcacatgaaatgcagtatactgatggtcctggagactgttgcagttgaatagggcagctactgggatgatggtgtttcccccggatgaggatgacaggaatgcagggcctaggatttgttgagcatgtacactcttcttctgaattggccacccagaaaccaattattgaatcagaacaacacaaattggtttgtgcttgagccaggtctgtagaaacggaaatcaattcagttgtggaaatgatgaattttaaaagctgctgggtttttttttgtgcaaggtagagattttcataacatctcaataatccttttgaaatgtgcagttgcttagtgcaaaaaaagaaatagtgccaccatttcttcaactaaaagataaggtgtgctttgtaaaagtaaagcatatccaattttcatcctgttggtcggtattaccaagggtcatgatgtagctggcgcacaaatgtgaagaatcatttactacttattttattgttttcgatctgcatgcacaatatgaaatcataaaagcaacaaacatcaccacaccaacactgagtaagatcatttctatcaggccaaggaggtttatttttccagttacttgacttctgaacatgtttgccttctcatcaccaatggtcccagtctcattaagccaaagaataggcacaatatagttcctcttcagattctttaatacttgaattttttctgatggcttgaccaataggttgacctgcagccgttttgcaaattgtaaagtgaatccagttataggttcaatatccaagtatgtcctatgttcttcttcatttgggtttaatccatcaataggttctgaaacatcaggacttgcatacagaaaatgaggaagtgaaatgtacacaggtctcccttctttgcatttgctgatgtctagcacaccatatgatgtacaattttttgagataattttttctgtgcagaaacaatagttgtctgggttttcaactggagaggcaaaggccttggatggaagaacaaatctatacacagggattcctttcagattaacgtcggattcaaatacagcatagattgacctgcaaatatcagaagaaaagaactgcaatacctggcttttctcaacaaaaggtggaaatgaggctgcatctgtaccattaatcatgtcgcagtgactttcccaataggacagattccttttacctttatatgtgtcgattatggcaactttacttatgttatcttttccattgaaaactttataaactccatctgcagtattgttgtaaggataaaacagaccaactgtggtagtaacagggtacggaaccaaactcaaaaatggatccctatagccccataacagttctctcaaagttctgacttggaacatagaagattttgacttgttaataagtgaattgaggatcatttgaacaaattgattttgatagatatgggatgcagctgccacagccagattgagaactgtgaagttgtcagcctctgttccaactgatagtgaaggttcgaagatggcaccattgggctgcaggaaagagactgtgttgtcctcagcgtcctgggttacattttccttggctagaaaacgaactctgtacgtataaggacctctttgcttaacttgaatgttgctgctgttcatcatcacttcctgtggattttgcacatcaaagatccaaaactgtctgtaaacttctgtgcctgttttaacccaatttttaaaagcaattgtaccttcttcgaggacaacttgctttttaattgtcttctggataagcaggtctccaactggcattagaatacctccaaacacagccaggacagcaccaatgacagccccagcgatgagcccacagttccggtcacagcccatttttcttgttcaggaggtgaattagtgttaagcacctgtttcttgcaaactcctggatatgattaaagtggtttctacaagctctggttcttattcacaaatcaacagcaagacatgaattttacaggaaatgaactgatgagtcacagaaagaatcaattcgtctaatcattggaaagctatctttaaaatggctaagaaggatttttcaatcaaatgctccaacatttggacaattcttaataggatcaaatggtattctgcaggaaagtcctacactgcagtcctc

SEQ ID NO: 13820 - RNA, 4005 nt, Homo sapiens
  source 1..4005: mol_type = other RNA
gctgggattacaggcatgagccaccatgcctggccatgtatacacatcttaatacaaatattttcagagataaccattgcgtgatagctattttttttcttgaaatgataccctccttcacccttttctgtcagaactgaaagctacatagcttcttctatttcttcatgcacttgttagaagcaatatgcattaacctattttccgatgctgttgattctctaatctgttaatccatttgcagacgctattgattttcaaacttaagttatgaatacctgctataattctgtggttaataaccagctttggaaagaaaatgtgcttctatcaaagggtacaatttttctatgactaaaacatataaattcatccatgagcaattgcaagtgtccaaacatttaccctttctgaacaacattaacttcgccagggcaaaacaaagtcacacatgtaacatattccccaagttgccccactcccaccacagtgcatatgtgcacacacacacacacacacacacacacacacatccaaagcccagatttcatgtaaaaaaaatctccccttaagtaattatttttcctactgcatatttttaatctcgttgtctttgtatatgaattgtctttcctcttatattccttttacagaatttgagaaatgaaacactgaggaatgataaagattatacatgtattcaaacaatattaaagacatataggtcaaaaccttttctgatatctaaatgctatgagatcatccctgtattaagatctgagtcatgattagtcataatatacaggtcaatatgtatattctcatccaattatctttagaagtttctacattatataactcagccctacatgcctcaatgattaaaaaactttcctttatattagatggacatgtccacaaatatcctaatgcaaatagaataaaccttgtattatcagaagaacatgtctacaatgttatcttacatattaatatcttggacagatacttcttttatcttcccagttaaaaggaaaggcactaagtatgctttaagcaccttcagagatgcaaaagatctttccaaacaggtagattcttggtttgtggcttttctgtagtaatgctcaacatttactctggcggctatcataaggaggaggctaaaagttattttcgattttagtatccaaacaggccagttactattcctttgtcctgtatccttctgtgggtaaaacacaagctagaatttggtttatcttccctttctatgctggagctttttaggagaactaatgctctcagaataagtgaacccctgctcaagaaacagagttacctattaatgtgtctccttatgaaaaaggaaaaacctttgcaattgtcctactgctgtaaaggatgaaaccaaatgtctttttgttcttcatccaattagcttaaaaaattagcctagaacaaagtggtagaaatttagaaagcatatttcagcaaggactatggatttataaagaaatgtggattcagataaaatatacttcagagagaaaattaggataaacattttatgacacaagaggaactagaaaaagcacaggaatttaaggaagaacatattttaatggttgaaacctgtctttatgaggcgattatgacagcaaaaaatattataatgaataacaatgcatagtctacgctttgtaatatttcatacaataattcctttatcatttacatctcttaatgctagaaaagcattctgaagatgccaagcgtaagttgcaactgagtaaaaaaaaaaaagcaaaatttactcaatttccagaagaggtgcagaacagagaatgaaggtccttaaaatataaaccgctagtgtgctaaaatgatgtccatttgcaggatcagtgacaaaatatttaagcccataaagaaaagagttatacctgctgtatgaaggtattcatagagaaatatgagtcataagccaattatttataaatgtctttcaaaatatttggtgcacatgaaatgcagtatactgatggtcctggagactgttgcagttgaatagggcagctactgggatgatggtgtttcccccggatgaggatgacaggaatgcagggcctaggatttgttgagcatgtacactcttcttctgaattggccacccagaaaccaattattgaatcagaacaacacaaattggtttgtgcttgagccaggtttattttattgttttcgatctgcatgcacaatatgaaatcataaaagcaacaaacatcaccacaccaacactgagtaagatcatttctatcaggccaaggaggtttatttttccagttacttgacttctgaacatgtttgccttctcatcaccaatggtcccagtctcattaagccaaagaataggcacaatatagttcctcttcagattctttaatacttgaattttttctgatggcttgaccaataggttgacctgcagccgttttgcaaattgtaaagtgaatccagttataggttcaatatccaagtatgtcctatgttcttcttcatttgggtttaatccatcaataggttctgaaacatcaggacttgcatacagaaaatgaggaagtgaaatgtacacaggtctcccttctttgcatttgctgatgtctagcacaccatatgatgtacaattttttgagataattttttctgtgcagaaacaatagttgtctgggttttcaactggagaggcaaaggccttggatggaagaacaaatctatacacagggattcctttcagattaacgtcggattcaaatacagcatagattgacctgcaaatatcagaagaaaagaactgcaatacctggcttttctcaacaaaaggtggaaatgaggctgcatctgtaccattaatcatgtcgcagtgactttcccaataggacagattccttttacctttatatgtgtcgattatggcaactttacttatgttatcttttccattgaaaactttataaactccatctgcagtattgttgtaaggataaaacagaccaactgtggtagtaacagggtacggaaccaaactcaaaaatggatccctatagccccataacagttctctcaaagttctgacttggaacatagaagattttgacttgttaataagtgaattgaggatcatttgaacaaattgattttgatagatatgggatgcagctgccacagccagattgagaactgtgaagttgtcagcctctgttccaactgatagtgaaggttcgaagatggcaccattgggctgcaggaaagagactgtgttgtcctcagcgtcctgggttacattttccttggctagaaaacgaactctgtacgtataaggacctctttgcttaacttgaatgttgctgctgttcatcatcacttcctgtggattttgcacatcaaagatccaaaactgtctgtaaacttctgtgcctgttttaacccaatttttaaaagcaattgtaccttcttcgaggacaacttgctttttaattgtcttctggataagcaggtctccaactggcattagaatacctccaaacacagccaggacagcaccaatgacagccccagcgatgagcccacagttccggtcacagcccatttttcttgttcaggaggtgaattagtgttaagcacctgtttcttgcaaactcctggatatgattaaagtggtttctacaagctctggttcttattcacaaatcaacagcaagacatgaattttacaggaaatgaactgatgagtcacagaaagaatcaattcgtctaatcattggaaagctatcaacttctagaagagcttgctttcggagatgtaggacctcaagactggctccagagtcttgcaggagcagatgcagaaagtaaacaggatttccacggcatagcagctgagaactcagaaatgaggcacaggctctcaacccttcatctatccttaaggttatcctgacatct

SEQ ID NO: 13821 - RNA, 3931 nt, Homo sapiens
  source 1..3931: mol_type = other RNA
gctgggattacaggcatgagccaccatgcctggccatgtatacacatcttaatacaaatattttcagagataaccattgcgtgatagctattttttttcttgaaatgataccctccttcacccttttctgtcagaactgaaagctacatagcttcttctatttcttcatgcacttgttagaagcaatatgcattaacctattttccgatgctgttgattctctaatctgttaatccatttgcagacgctattgattttcaaacttaagttatgaatacctgctataattctgtggttaataaccagctttggaaagaaaatgtgcttctatcaaagggtacaatttttctatgactaaaacatataaattcatccatgagcaattgcaagtgtccaaacatttaccctttctgaacaacattaacttcgccagggcaaaacaaagtcacacatgtaacatattccccaagttgccccactcccaccacagtgcatatgtgcacacacacacacacacacacacacacacacatccaaagcccagatttcatgtaaaaaaaatctccccttaagtaattatttttcctactgcatatttttaatctcgttgtctttgtatatgaattgtctttcctcttatattccttttacagaatttgagaaatgaaacactgaggaatgataaagattatacatgtattcaaacaatattaaagacatataggtcaaaaccttttctgatatctaaatgctatgagatcatccctgtattaagatctgagtcatgattagtcataatatacaggtcaatatgtatattctcatccaattatctttagaagtttctacattatataactcagccctacatgcctcaatgattaaaaaactttcctttatattagatggacatgtccacaaatatcctaatgcaaatagaataaaccttgtattatcagaagaacatgtctacaatgttatcttacatattaatatcttggacagatacttcttttatcttcccagttaaaaggaaaggcactaagtatgctttaagcaccttcagagatgcaaaagatctttccaaacaggtagattcttggtttgtggcttttctgtagtaatgctcaacatttactctggcggctatcataaggaggaggctaaaagttattttcgattttagtatccaaacaggccagttactattcctttgtcctgtatccttctgtgggtaaaacacaagctagaatttggtttatcttccctttctatgctggagctttttaggagaactaatgctctcagaataagtgaacccctgctcaagaaacagagttacctattaatgtgtctccttatgaaaaaggaaaaacctttgcaattgtcctactgctgtaaaggatgaaaccaaatgtctttttgttcttcatccaattagcttaaaaaattagcctagaacaaagtggtagaaatttagaaagcatatttcagcaaggactatggatttataaagaaatgtggattcagataaaatatacttcagagagaaaattaggataaacattttatgacacaagaggaactagaaaaagcacaggaatttaaggaagaacatattttaatggttgaaacctgtctttatgaggcgattatgacagcaaaaaatattataatgaataacaatgcatagtctacgctttgtaatatttcatacaataattcctttatcatttacatctcttaatgctagaaaagcattctgaagatgccaagcgtaagttgcaactgagtaaaaaaaaaaaagcaaaatttactcaatttccagaagaggtgcagaacagagaatgaaggtccttaaaatataaaccgctagtgtgctaaaatgatgtccatttgcaggatcagtgacaaaatatttaagcccataaagaaaagagttatacctgctgtatgaaggtattcatagagaaatatgagtcataagccaattatttataaatgtctttcaaaatatttggtgcacatgaaatgcagtatactgatggtcctggagactgttgcagttgaatagggcagctactgggatgatggtgtttcccccggatgaggatgacaggaatgcagggcctaggatttgttgagcatgtacactcttcttctgaattggccacccagaaaccaattattgaatcagaacaacacaaattggtttgtgcttgagccaggtttattttattgttttcgatctgcatgcacaatatgaaatcataaaagcaacaaacatcaccacaccaacactgagtaagatcatttctatcaggccaaggaggtttatttttccagttacttgacttctgaacatgtttgccttctcatcaccaatggtcccagtctcattaagccaaagaataggcacaatatagttcctcttcagattctttaatacttgaattttttctgatggcttgaccaataggttgacctgcagccgttttgcaaattgtaaagtgaatccagttataggttcaatatccaagtatgtcctatgttcttcttcatttgggtttaatccatcaataggttctgaaacatcaggacttgcatacagaaaatgaggaagtgaaatgtacacaggtctcccttctttgcatttgctgatgtctagcacaccatatgatgtacaattttttgagataattttttctgtgcagaaacaatagttgtctgggttttcaactggagaggcaaaggccttggatggaagaacaaatctatacacagggattcctttcagattaacgtcggattcaaatacagcatagattgacctgcaaatatcagaagaaaagaactgcaatacctggcttttctcaacaaaaggtggaaatgaggctgcatctgtaccattaatcatgtcgcagtgactttcccaataggacagattccttttacctttatatgtgtcgattatggcaactttacttatgttatcttttccattgaaaactttataaactccatctgcagtattgttgtaaggataaaacagaccaactgtggtagtaacagggtacggaaccaaactcaaaaatggatccctatagccccataacagttctctcaaagttctgacttggaacatagaagattttgacttgttaataagtgaattgaggatcatttgaacaaattgattttgatagatatgggatgcagctgccacagccagattgagaactgtgaagttgtcagcctctgttccaactgatagtgaaggttcgaagatggcaccattgggctgcaggaaagagactgtgttgtcctcagcgtcctgggttacattttccttggctagaaaacgaactctgtacgtataaggacctctttgcttaacttgaatgttgctgctgttcatcatcacttcctgtggattttgcacatcaaagatccaaaactgtctgtaaacttctgtgcctgttttaacccaatttttaaaagcaattgtaccttcttcgaggacaacttgctttttaattgtcttctggataagcaggtctccaactggcattagaatacctccaaacacagccaggacagcaccaatgacagccccagcgatgagcccacagttccggtcacagcccatttttcttgttcaggaggtgaattagtgttaagcacctgtttcttgcaaactcctggatatgattaaagtggtttctacaagctctggttcttattcacaaatcaacagcaagacatgaattttacaggaaatgaactgatgagtcacagaaagaatcaattcgtctaatcattggaaagctatcattagaagtccgatgaaagagcacaaggccacaaatgttaatgcactttcagaatgctagttgggaagaccagggaattaacaccgaagactctggtt

SEQ ID NO: 13822 - RNA, 3937 nt, Homo sapiens
  source 1..3937: mol_type = other RNA
gctgggattacaggcatgagccaccatgcctggccatgtatacacatcttaatacaaatattttcagagataaccattgcgtgatagctattttttttcttgaaatgataccctccttcacccttttctgtcagaactgaaagctacatagcttcttctatttcttcatgcacttgttagaagcaatatgcattaacctattttccgatgctgttgattctctaatctgttaatccatttgcagacgctattgattttcaaacttaagttatgaatacctgctataattctgtggttaataaccagctttggaaagaaaatgtgcttctatcaaagggtacaatttttctatgactaaaacatataaattcatccatgagcaattgcaagtgtccaaacatttaccctttctgaacaacattaacttcgccagggcaaaacaaagtcacacatgtaacatattccccaagttgccccactcccaccacagtgcatatgtgcacacacacacacacacacacacacacacacatccaaagcccagatttcatgtaaaaaaaatctccccttaagtaattatttttcctactgcatatttttaatctcgttgtctttgtatatgaattgtctttcctcttatattccttttacagaatttgagaaatgaaacactgaggaatgataaagattatacatgtattcaaacaatattaaagacatataggtcaaaaccttttctgatatctaaatgctatgagatcatccctgtattaagatctgagtcatgattagtcataatatacaggtcaatatgtatattctcatccaattatctttagaagtttctacattatataactcagccctacatgcctcaatgattaaaaaactttcctttatattagatggacatgtccacaaatatcctaatgcaaatagaataaaccttgtattatcagaagaacatgtctacaatgttatcttacatattaatatcttggacagatacttcttttatcttcccagttaaaaggaaaggcactaagtatgctttaagcaccttcagagatgcaaaagatctttccaaacaggtagattcttggtttgtggcttttctgtagtaatgctcaacatttactctggcggctatcataaggaggaggctaaaagttattttcgattttagtatccaaacaggccagttactattcctttgtcctgtatccttctgtgggtaaaacacaagctagaatttggtttatcttccctttctatgctggagctttttaggagaactaatgctctcagaataagtgaacccctgctcaagaaacagagttacctattaatgtgtctccttatgaaaaaggaaaaacctttgcaattgtcctactgctgtaaaggatgaaaccaaatgtctttttgttcttcatccaattagcttaaaaaattagcctagaacaaagtggtagaaatttagaaagcatatttcagcaaggactatggatttataaagaaatgtggattcagataaaatatacttcagagagaaaattaggataaacattttatgacacaagaggaactagaaaaagcacaggaatttaaggaagaacatattttaatggttgaaacctgtctttatgaggcgattatgacagcaaaaaatattataatgaataacaatgcatagtctacgctttgtaatatttcatacaataattcctttatcatttacatctcttaatgctagaaaagcattctgaagatgccaagcgtaagttgcaactgagtaaaaaaaaaaaagcaaaatttactcaatttccagaagaggtgcagaacagagaatgaaggtccttaaaatataaaccgctagtgtgctaaaatgatgtccatttgcaggatcagtgacaaaatatttaagcccataaagaaaagagttatacctgctgtatgaaggtattcatagagaaatatgagtcataagccaattatttataaatgtctttcaaaatatttggtgcacatgaaatgcagtatactgatggtcctggagactgttgcagttgaatagggcagctactgggatgatggtgtttcccccggatgaggatgacaggaatgcagggcctaggatttgttgagcatgtacactcttcttctgaattggccacccagaaaccaattattgaatcagaacaacacaaattggtttgtgcttgagccaggtttattttattgttttcgatctgcatgcacaatatgaaatcataaaagcaacaaacatcaccacaccaacactgagtaagatcatttctatcaggccaaggaggtttatttttccagttacttgacttctgaacatgtttgccttctcatcaccaatggtcccagtctcattaagccaaagaataggcacaatatagttcctcttcagattctttaatacttgaattttttctgatggcttgaccaataggttgacctgcagccgttttgcaaattgtaaagtgaatccagttataggttcaatatccaagtatgtcctatgttcttcttcatttgggtttaatccatcaataggttctgaaacatcaggacttgcatacagaaaatgaggaagtgaaatgtacacaggtctcccttctttgcatttgctgatgtctagcacaccatatgatgtacaattttttgagataattttttctgtgcagaaacaatagttgtctgggttttcaactggagaggcaaaggccttggatggaagaacaaatctatacacagggattcctttcagattaacgtcggattcaaatacagcatagattgacctgcaaatatcagaagaaaagaactgcaatacctggcttttctcaacaaaaggtggaaatgaggctgcatctgtaccattaatcatgtcgcagtgactttcccaataggacagattccttttacctttatatgtgtcgattatggcaactttacttatgttatcttttccattgaaaactttataaactccatctgcagtattgttgtaaggataaaacagaccaactgtggtagtaacagggtacggaaccaaactcaaaaatggatccctatagccccataacagttctctcaaagttctgacttggaacatagaagattttgacttgttaataagtgaattgaggatcatttgaacaaattgattttgatagatatgggatgcagctgccacagccagattgagaactgtgaagttgtcagcctctgttccaactgatagtgaaggttcgaagatggcaccattgggctgcaggaaagagactgtgttgtcctcagcgtcctgggttacattttccttggctagaaaacgaactctgtacgtataaggacctctttgcttaacttgaatgttgctgctgttcatcatcacttcctgtggattttgcacatcaaagatccaaaactgtctgtaaacttctgtgcctgttttaacccaatttttaaaagcaattgtaccttcttcgaggacaacttgctttttaattgtcttctggataagcaggtctccaactggcattagaatacctccaaacacagccaggacagcaccaatgacagccccagcgatgagcccacagttccggtcacagcccatttttcttgttcaggaggtgaattagtgttaagcacctgtttcttgcaaactcctggatatgattaaagtggtttctacaagctctggttcttattcacaaatcaacagcaagacatgaattttacaggaaatgaactgatgagtcacagaaagaatcaattcgtctaatcattggaaagctatctttaaaatggctaagaaggatttttcaatcaaatgctccaacatttggacaattcttaataggatcaaatggtattctgcaggaaagtcctacactgcagtcct

SEQ ID NO: 13823 - RNA, 2152 nt, Homo sapiens
  source 1..2152: mol_type = other RNA
gctgggattacaggcatgagccaccatgcctggcccagattctttttgataaaggatatttctgagtggatctcctgaatggatctatctgggagtgccttgagcaaaatcactgctataggtacgtcaactagttatgtcccttataattaatacaattattaattcatacagagtataagtcaaaatcttataaaattggttaatattggttatcattcagcaaatatttattgagtatctactgtatggcaggctgggctacaggcgggggatgtaatagtgaaaaaggcagaaatggtcctttaattgccgtctgatgatgattataggcctaagtgacccgcgctcaactgatgcgacctaattcctgagcctgttaaactgcagggtaaatcatgggctgaacagtcactcagtgaagtcttatctgaaatagccaggcagtttgcccctccattataacccttagattgcctgcttttgctcttcctccttcagcaacttcatcagctcttccagctggaccatcagctcccgcctgctctcctgcagggccgacatcctctgctccagttcatccttcctttgcctcagcagccgcagctctgccagcagcgtggggttctgctgtgccttctcaggggtgggctgggaggcctgctcgtgttccaggcggagacgctgaatctcctgcaggatctctctgtttttgttttccagttctgcaataagctgtctttgttgtttgttggcatcaaagttaaagctcaagtcagtgggaggacgagtcacgtttcctgcttctgcagccagccgggcagcatagcgagctataagacggtgttcctcatccagtcggctaggactgtccagaacactcttggtgggagtgggcactccagaggacatgtggctaaccatggtgtcattcatattagtcagagggcgaggaggaactatatgtgcaaggtcaagtggtttctctggttgctcaggaaaaacaggatgcgggggttctctcgtgggtacacaccccaaagatttactaattgcatggctcagcttctttgcaggagatttccaagaggaatgctccttcatctggtgctggttgctgtgagggccgccggcatggccacgccaaaagcaattctggcagagctgatagttgtggcactgctggcatcggtaccggaaacccatcatactctcacatcggcagtaggagcactccacgggatggaagacattctcaacatgggcaagcctgtgcatgagaggtagccagacaaggcactggggaggagggtcagccatcattgtgtctaaaaacatatttagcattatctttctctgctgtggaaaacaggtgcggactgagtgctctgtgtaaccaaaagatggcccttcaaagacagctgttgggagcttcagaacttccttcagaaactggtcaaacttgctaaatatcattaagccattggaatctgacatctgggagaaaacatatctcaatttgtccagcatttttccaccacacatggttgctaacatagctttaactgaaaataccgtcaacttgcctcggccctcactgtcatatgcagcaatcataaagttgaggaggaggctgatagattgttccacactaatttggtgagtagaaggaaggcgcttgttcaactgatagtagatggaggagatgacagtttcgaggcgggacacactgatctcggtggtatggtccagtgtattaaggccattgtctcggaaggcttcaatcatgttccagatatcaacaagatgaaggttgcatcgtttttgtacaaatcgtaatttgcaggctgttctgtaagttgatagtcgtatgacatcaaaattctgagcacgcatttctatgaacagctgcctcttctctgccatggtcttccgcttgttcccactttcctcaatcatccttgctcacttccccgccggagcaggggtcgtcgggaaggtctcctgcggcctcactcctccgcacgctccggcccagccccctcggctgaggcagcggcagcgcctactcaggccccggagccacccccgcggcgaacgttcgcagcgcccggctcgcgccgcttctccgcccggcacgcgcagcgcccgc

SEQ ID NO: 13824 - RNA, 1525 nt, Homo sapiens
  source 1..1525: mol_type = other RNA
gctgggattacaggcatgagccaccatgcctggcccctaaattcttttttgttgttttgtttttgagacagtctcgctctgtcacccaggctggagtacagtggcacaatctcagctcactgcaacttccgcctccctggttcaagcaattcttctgcttcagcctcctgagtagctgggactacaggcatgcaccaccacgcctggctaattttattttttttgtatttttagtagagacagggtttcaccatgttggccaggcttgtcttcaactcctgacctcatgatccgactgcctcagcctcccaaagtgctgggattacaggtgtgagccactgtgcccgggcttttttttttttttttttttttgagatggagtttcactctttcccccaggctggagtacagtagtacagtagtgtgatctcagctcactgcaacctctgctttccaatttcaagcgattcctgcctcagcctccagaatagctgggattataggcgcccaccaccatgcccagctaatttttctattttcagtggagacggggtttcacatgttggccaggctggtcttgaattcctgacctcgtgatctacctgcctcgacctcccaaagtgctgggattagaggtgtgagccacagcacccagccaaattatttttttttaatcactcaaaatcaagcatgttgtaggtaccaaaattctaactcaaggtggcctatgaactgggttcataacctacatctatctatatatatagtggctcctaggcaggtagctggccttttagatattcataagctgtcttggagacacatgccatttgagtacagtaactctgctgagactccagatgtaccttgaatactgttgagagctagtcagatgaatgagactggcctgccacctagcatctgcacatgaggtattcttctacactgatttttcatacaggtgtgctagattttaatgggtcacttaaattcagttagtctccaacatataaattctccacaacataggatatagtatacactctacttgacccaagatgataaaactgaaaaagacaaaaaaaaattttattgccataaattaatccagtaggtatatttgagaaagcacgcatcagttggttagggcaataagcgcctctaccacgttgcccatgtgttcccgcaaactgcgttctgctgctgctcgagatatctccatctcagtcattattagctccagatcttccttcttgatagtgacttttgccagttctttctcccgctcctgtttggctttctgctcccgggaccttctgtctccaatcacagacatggccgtctccagattggaactctggatctccttctcctctgcatagtcggtgacccgctccaagtccgccgcaccgctgtcatgtttccgtggcttctccggaggccgctctggtccactggtctcagtctccaactccagctccacatccccctcggtcgccatatctatttcaccacgccgccgcat

SEQ ID NO: 13825 - RNA, 2667 nt, Homo sapiens
  source 1..2667: mol_type = other RNA
gctgggattacaggcatgagccaccatgcctggcctaactacttcaaatttatactccttgtctctgattggcttcccttagcactcttcagcgtacagtttttcagaaaggttgagataaacacaatattcatagatttcctgccttcacatctgtttaagggtggtttccaatctttgcagaagtgttcatctatgtcaattctaagggtagacaataggtccaatgtggccatccatctcatggaaaatgcagccacactctttatagtatctaactcagcagaggcagcattcgggatgtttcatgttaattcccaagaaagagtctggtatttgtttcacttcaaatacattcttctctgttaccatcacaaaagcagcgagactccttgggggtgaatcccaatcaaagcaactattaacgtagtatgcagcatttaccagcaccatgacacaacgtttcattctgataaagtttcttagtagcagctgtttagagagtctgttttcctcttcaatgtacttctgttctttgggtattaatgttcgtaagctggctttcacagcattaaaaatcacatctatttcaagatagatgaccccctttgttggccctgtcagctgcttgtttttcaagacgtaggctttctgttcaccattttgaatagacagcaatggtatagcaactttgcccagaaagtcagcacttcgatcccgatcttcatcataaactgtcacttcaagaactgaatggatatctttaatgttgaacgtgaagactttattccactcaggattgagatttttgtagacagtatgtgttagcagtctatcgttgttcagttctaccacacaaaatgggtcactttttccagtgacgtcggcagccattaacccttccgctctgatgactttcacctggagaaatcccacatctttcaggttgtgaaatatcctcaatgggctatatctctttaatatctcctctcgttccttctggtcctccagggagttgacagacaggtcagagatgctgactgtggctgatgctgtcagagtgaccagcagcaccaggtgtccctcaccctcttccagctgcaactccagcttgtgcgtctgttccctactgagggctgacaggtcgacctggcacctgccaatgaaatcatcccttttcccagcatctttgtcccatgcagtgatatcaatgactcctcctctttcttcataaaggtgaaaatcaaattgttccctccactgaggattcaacgtttttggcataatcttgctcttgtacttctgatgcccaagccggaacttcacgtagggatcgctcaacccgttggaatccatggccttgaggtctctcccttcaatcaaggtgatgctgactattcctctccaaagatgcgattttctgtgtaggtctgataggcgtaaactttgggtctgaaacttacttgatcttttccaactcttcctcattagcattgtcacatccctggactctccttctttaggggtaaggatgactgagagcaaaatgattccaagatcatggtcaggataatgaggatctttcagagtaagggtcacatctgtgggcctgtttaactccaattgtgtcagatccagaaaggctgagcccataaagtcatcctgtagtccaaaatcatagtcaaatacctttatatacaatggctccctaagatgatcaaccagaatacaagctttttcttcccacacagggttgaggttcttgtgtattatcttacttctaaaaacttcttttcctccgattttaaacttcacatatggatcactcgtccctcctcgatctcgagcagctaaactttgaccccttcttaatgtaatgtccagctggtacattccgggatcagccaaggggacttctgcattactggttccagcagtgtttattattttctggctgctgccgtgctcctcgcccgtctccggggcccgagactccgcgggactccgcgccggctctgcgggaggaggcggcggctccagcagctgctccaggcaggcggtgcccggcagagaggagctcttctggtggcacaagtgcgccccggggccctgacgccgtgcaccctcatctcgggcgcggtcccccctcgggggaggctggggcgaggaggacagggaggatgaggcggaggaagaggaaggagctgagtcgggggagcgtccgccaggaggcgtccctcccgctgctcccgaggccgccgcgggcccctttacggcggggagcaaatgctcgcggatccggcggcgtagcgtggacccctgctcggctctgccggcgccgccgggctccaggggctccggcgacgagcagcacaggttgggctgcgaggaggagaagactcggtccagcacttgcttccgcttcttgaagccgctccacctgctgcctgcaccactccccctggccggtgcattccctgtgcccaccgggggtggcggggagggcgacggggtgtccgcagtgcggcgctctggacccccagcgcgcccgcccccgccgcccttgctcctgcccacccccagctgcaggttcttccagagccgggcctggaaggaggaggacgccgccggcggctctggctcgcccgccgcggcagcccggggctc

SEQ ID NO: 13826 - RNA, 7079 nt, Homo sapiens
  source 1..7079: mol_type = other RNA
gctgggattacaggcatgagccaccatgcctggcctactagaaatatttttaaaagttatattctcataaacaattaaaatttcattccttcatttaaaaatgttttgtaaggaagaataaagacaagaatgtgtaataatatattttagatatgcagaaagtctacttaatttttaggttagacaattttatacaaagcaggcccctttttgaattggtattgtttcgtttatttaaagaattatatggatcaaaagagggcaattaagaattatgaattatgaattctttttcatagacacagaaattaaaagaacttttccttagaaagatgcataattcacctctactcttagtaaataaaacattttagtaaacaaatatcttatcctcaaatacacttttattctaaatattgatattaattacatagaaattcacatagaagctattcattcctcatatcttatagtgctttatttttaaatttataaatgtttttcaatctatcactgccaaatgagcaatttagcacacaaacatgtacttattttatttaaaaaaaaatggagttgagaataatttatatatacatatgtatactgacatttataaaattgtaaatcatactggaaaaatactatacatattattctcagtatgcaaagtaggagaaaaacacctaaaacctttaatcagtcttaaaattctgatagttttacaaattagttctaatccgtagcaatgggaccatttctttttcttttctttgagacagaatcttgctctgtcacccaggatgcagtgcagtggcacaatcttggctcactgcaactgccgcctcctgggttcaagtgattcttgggcctcagccccccgagtaggtgggattacaggtgtgtactaccacacctggctaatttttgcatttttgtaaaaatggggtttcaccatgttggccaggctggtctcaaactcccgagctcaggcaatccaccagccgtggactcccaaagtgttgggaagtaagccactgtgcctggctgggaccacttctaatatgaggcttacaaggtagaatttatatgctgctgggacaaaagctaagtggcaaatatgacatcagatgatctaactgaccttctcagcagatactctgcatcacttgtaaaacaaaagaaagtcaaacacagtgttttttttttttacataattttcagttaactttaaatacaagatacacatgtgttaaattattactaatctaccagattattgtttaacttgttgaatacctataatctctgctttttctgaaagctggcatttattaaacatgtggagttttcacatgttcctggcattatttataatttgaggtgtttcaccgacatcagagtaatacattgcttactctccactgatttgtacactggaaaaatgttgtttgctgcagtgtagtagctacatatcattctttagtcctttacatgcagaccaaagaaatgaaaactggctgggcatggtggcttatgcctataatcccaacatgttgggaggctgaggtgggcggatcacttgagcccaggagtttgagactagcttggccaacatggcgaaaccctgtctctactaaaaatacaaaaattagttgtgcatgcagttgtgcacgcctgtaatcccagctacttgggaggctggggcaggaggatcgcctgagcctgggaggtggaggctgcagtgagccaagatcatgccactgcactccagccagggcaacagagcaaaacactatcttaaaaaaaaaaaaaaaggaaatgggaaactgttaagaatatgcttttcataaaagtccagttacttatttacaaaatactaaaggccaatgataaggtgatatgaactgaggagtaccattacccaagccttctgtacctgaagtccaattgtaaaaaaaaccccaaagcccatccacctttgtcttaaacaggtctacattgtacttctaaacttgtacagtcttcatgaaattaacatcttcatgttttcttaagcactttggtttagaaacttcttaaaatatcattcaaaaagagcttagagcatgtacagagttcatataaagctctattttacataattgtatatactgctatctcaggaacatgatatgttatttagaaaagatagtagggcaaaaaaacaaaacacaaggtccaggtacaaataattccagccagttatggtggctcacacctgtaatcccaggacttttggaggctgtggtgggaggattgcttgaacctagaagttcaaaaccagcctgagcaacacggtgaaaccctatctgtacaaaagatacaaaaaattagccagtcctagtagtgcacaccagtagtcccagctacttgggaggctgaggtaatagaatcacctgagcctgggaagttgaggctgcagtgagccataatcacaccattgcactccagcctgggcatcagcatgagaccccgtctcaaaaaaagaaaaataaaaaaaaacacccaaaaactatccccaagaggactaagaaggaaataaaactttggtgccagacaagacagtatcaagataaagccaaagagttgctaaaaacaaaaaataataataattcaggcaattggttgtctgggttctgcaatttgaaatattccactagacactaatatacaggaactcttttggtcattgtcacatagcagaaatgctgctatatgtgaagttgttctggactgcctgttatagctattaaatggaaaccccagaattcatcctgaatgtctctgaatgtgaaaagtcacatgcgttaatttaattcagtataaaatttccatgttctcccacaaggaggatttcagcagtgtcttcccagcatgaaaccatgtcttatcactccaccagattcagaattggtactaattctgacagaagctgaaactaaagcctatgttttctttagtcaacataaggccttttttcagagatggtgtgaattaatagtttaaaccaccaaaataaaagaatagacaagtattttcttaacatatccatttccattgctagagctgcggtgatcagcagaagcatctgcctggctgtcaatatcaaggtggatccaggctgttggaactggtggatccaggggttggaacggaggaatactaaaaatgagacttggaacttggaaggcctacaccacgagggccaattctgccataagccctattgcccagatatgttacataaaacatccagatattacagtgaaagtcagtgtgtggccagacacagtggctcacaattgtaatccagcactttgggaggccgaggctggtggatcacttgaggtcaggagtttgagaccagcctgaccaacatggtgaaaaccccatctctactaaaaatacaaaaattagctgggcatagtgacacaggcctgtaatctcagttgcttgggaggctgaggcaagagaattgcttgaacctgggaggcggaggttgcagtgagccgagatcgtgacactgcactctaacctgggtgacagagtgagactccatctcaaaaaaaaaaaaaaaaagtcaggtgagaagaagtagcacatagtgaaaatgaatataataattttacagctggtcgggctcagtggctcatgcctgtaatcccagcactttgggaggctgagacaggaggactgcttgagcccaggagtttgaaaccagcctgggcaacatagtgagaccctgtctttaaaaaataaaataaaataattttacagcttttggttctcctgtattatacagcataactaggagaaaaaaaaactatgaaattattttcccaagaccagttttactcatctttatcacatttgtttgatgtgggttatccaggagccacctacatcaaggtggatccaggctgtggtcttgcattgggtaacaaagcccttcccagagggaggagtcacaccattgggtcaagagtcatgaatgggtatttttacatatttattaaaacaagtttcctgagaagtttgactaggctatgttgttgttaacctagtttgcttaaaatgtacgaaaatgcaatcaaacttacatatcttttaaatattcgaaagtcagattttgttctgattgccctatccaattagggcaaattagtgagggtttttttggtttttgttttgtttttttaacaatagtctgaaacataaaattaagtttgggtttaaaaacaattcttgaaactgtcataaacatatgatatctattgattaaacagtaataaaaagacacaaggtacaagaattgaggcttggctgttctggctgtatactaacttcatataccctgacagaataaactatctttttaaaaagtgctttgtacactgcacaattatagctttaccaaataaaaactcaatgacatgtcgctgaaatttgcttcttctagaatttgaaattatttaaaatactgcatgagaatatttttatcatattatataatatgacttcatcaacatgaagttccaggaccccagatgcctctctgagaagttcattatttgatagggttggatcaaatgtaaaggcccaggtgttcaaagatcttagatacctaaagagagaaaggggcaaatggaggctcttctgagagtcaaaatgttgatgagaaacaaactgaaagtagcacacataggcagaaaaatagacaagttatgattcagaaaacaattgtatgcaattttggcataaatatctgagagtcactgtgggccatgagttgaaaaggaacatgcaagagagcaaggaaaacacaaagcctcattcagatgtgctggtgagaatatgacagaaaatctgttgaagttgtgtaccatgaagtctgtcttttgtcaaagttctatgcagtcccaggatagcgtgatagcagtggttaaacacaaccagctagttatagctttcattgtatggaaagacctctctggtctggaactctgcctttgaaattatccacgtagttcagaaggcaaatacttgttaaagggatcccaaaaggtaggagacaagtagtttttgttatgcattagggcagactttcaagcacaagacacaaaattgagcagcaaatgtttgggtagtcccatctcccttcggtttatatgtgggtagtaaaataaataaaattttccttctttgtctctttcttgaaataaaatatcaggtatccaaggagagctgaggattctcaatttgctagattgctttaaaggggtcagatttagaaaattaaggaataaatgaagaacaattttactggagtaggtgtggtcaataggcccttttccattttgtgccattgcttttagcacaaggatgtcaaaaatatcacatagaatgtcatctctgatggactgacagagacctcctgttgtgctgtgttaggacatgaggcttatcccagcttggcgggagagaatgctaagcatgatgagtgagatctgccacaggcacggatatttcctgctcctcttctgtttgtttcaaaccaccttcaggatctctgaaacatagaaggctgacagatgactcccacctgcacatacttcctacctacatgtcacatccaagggaggtatggtgaaacaagtgtgagctttgcagaaatgctgacaagcaagggaatttcagctgaggagaacattagttctttcactgaagattcctagtttctctgagaagttcttaagggtgaccagacctggccatgctagggtctacaagttaccaaacgccacctcatcaggactgtggacccctctcactgtgtcttcttggcaggcagagcttactgaccccctgggatggtgtattcattaaaatacttgctgtgtttggtgtcttttccatgacataacactcctcgagaaaagttcctgctgaatgtagtttacctgtcccacgacttgaataatcagaggaaattatccaaagctggttactgacccaaaaggaaaccatcgataaaacagcttcctgatttaggccctaaggaatgaagcagaaaggtgacgaacatttatcatgaccagagtgagttcagtgagctagaagttggctgagaggaggcaacacatgttgatcagaagtgagcacatcacccgcctccttctccaccctcagaggcagcgatggatggcagccaggccttttcctagtacttctcaattgcacattcttccaagtgcaagtgatgccatcattaggaagagtgggcgttggaagaaacagcaaaaggttcttgtgtctatgttgatttgaaattaattaaatttgtatcctcttcatcctctgttggcagcctcagcagactccctcaggggctgcttctcttggaaaacatgagcgccattcaggtttaggattcactgtcacttgggttgtgatttgattccttctcttccttcaaggtaggtaaacattcaaagtcggcatttctattcatgctgttcatccatttatcaagctcttccatttcaatttccataacagagggtgtatcttcctcaaaaatagggactttcacgttttcacttcccagttcatatgtctgtaaagcactctgagatccttggctagaaggttcttgtttagttctttttcttttatagtatgttgcaaggaataccacggataaaagtaagaggaccaataaaatcaatgggattaacaccatcagtataaactctaactgattttcatccggagcaaagttggtagaatttatatttgcatttaatgtttctttgatggtcactgcagcaaatgtgcttggaatagtcactttatttggtctttcagattccacagttgtatctcctgagttttctaattcctcataattaccccggccgacgggaacgagcgcgatcaccagggcgaagactagggctgcgcggggagcctgcatgtccgctcgcctcggcagaggcgcgctcaggatgctgcgccgggctgcagcctctctgaaacgt

SEQ ID NO: 13827 - RNA, 2358 nt, Homo sapiens
  source 1..2358: mol_type = other RNA
gctgggattacaggcatgagccaccatgcctggcctagactttatctttatatggcagttttaggttcacagcaaaattgagaaggtatggagatttccctaccctgttcccccacacaggcacagctgcccccatgggtatccctacctggagtggtgcatagaactggaatttgaacccagcgcccacagtccttcattcctatgacaccacttcacatgagtcaccacatctcagaactgctcagtcagctgaggcacagatggtgccacaggcccagagtgtgggtgactgcaggtgcctcagccccctggctggaaacagctagccacacacaaatggcagattgggagtcctcataggaaaaagttgtccctcttcagtctctttccttagaagcagagcctgagacaaggattcttgtgcaaatgctttactgagggagtactttctggagaaacctgtgagggaaccaggaaaactggataggccaaggggtcagaccaagcagagaggtggttccaggagaggcctggcctcagcccgatcccaggaacaatttgagagtgtcattcaacccagacaatcctgcacagacacgggggagctggcaattgtaccctccatggtgtcactctcctggccatgagtgacaggtggcctcttggtgggagaggtggggcagggggaaggcagctcccactagaccagggcagtatttaggggaaggaggcagattggagcagttggctgccaacacctggcctcactcagggagaggggccttgggcctggatgatatctgggtgaggtacccacaccatctgctgcaacctctgtgtatccattatgggctcacgccattcacaggcatgaattgagcacctagtatgtgggaaaacaggggaaacagagatggcacagacatggtctccatccttcgggggctccagtctagttgggggagatcagagaagttccatttgccactctaggccaagctaggtaagcggcagagccatgaagcattgtgggagcttggaggagggagtgagcccttgcagtcagggagaaggagtcagcctggggagacttccagaaagtagccctttgaccctgaggaggtggggatcagtcgtgatgaaagtaatagccattcagtagccccttgtaattcaccctgagccaatgcctggaggcaggagaaagtactcaaggctctggtgcctggagccacaagacctggcggctttgtctaggcttcacccaagaaggatttatggagctccttcttggttctggtgttgctttgggcaccagggatgcaactgagtttaagacaggcatggcctccacctgcagggacttcagagcttgcctggggagagggtcacatggccagactgtgcagggtccccagtgcctatgagaggctttatcttaggacagtggagggccttgaggttttaaaagatagagccacatggacagaaagatcaatattgccctttatagtggctgctgcggttgtagctccgagactatattggagggggtgaggaaggacaagggggccagcaggtgggggacagcggcagacccctcccccaccccgatgctttggtccaaacaccacctctgagggctcccttgcttgggcttctcccaagattcccatccaccctcagaggacacagctactgcctcaactgggaggattcggaaagcttcagaaggtcagaaggcattggtagagggttccgggggaggctgggactacctccccccggagtgtttgaaaagccaggctggttcaggttagatactgaggtggggatgccagagctccatgctgaggaacagggtagagggtgtgggcttctagcacccaggggtctgcccccggcagtggggccgccagtagaaacgcagtcgcttctggtaggtgtccaggttgcgcttcaggcagaaggccacctccttgtcacaggcacacagctgctgctcacaccagcttcccttgtcagagcagtggatgttcccctgggaaaagttgtatctgtaatagtccttgtagatgctgcacccctgggtcttcaggtggtcatagcagcagtcatgggtctggcagcaccagtccgtggcatctttgggttggcctctgccacctagtccgcagtgacagccgtagggccagtaggagaggatgggcattttcccagtcacttgcttgaccatcttgttcaggttcaggatcccgccctggattggaatcacaccagccatcaccaccagcccacacagcagtgcaagttccatgatcccagcacagagcagtggaggcagatgctggcagt

SEQ ID NO: 13828 - RNA, 2251 nt, Homo sapiens
  source 1..2251: mol_type = other RNA
gctgggattacaggcatgagccaccatgcctggcctagactttatctttatatggcagttttaggttcacagcaaaattgagaaggtatggagatttccctaccctgttcccccacacaggcacagctgcccccatgggtatccctacctggagtggtgcatagaactggaatttgaacccagcgcccacagtccttcattcctatgacaccacttcacatgagtcaccacatctcagaactgctcagtcagctgaggcacagatggtgccacaggcccagagtgtgggtgactgcaggtgcctcagccccctggctggaaacagctagccacacacaaatggcagattgggagtcctcataggaaaaagttgtccctcttcagtctctttccttagaagcagagcctgagacaaggattcttgtgcaaatgctttactgagggagtactttctggagaaacctgtgagggaaccaggaaaactggataggccaaggggtcagaccaagcagagaggtggttccaggagaggcctggcctcagcccgatcccaggaacaatttgagagtgtcattcaacccagacaatcctgcacagacacgggggagctggcaattgtaccctccatggtgtcactctcctggccatgagtgacaggtggcctcttggtgggagaggtggggcagggggaaggcagctcccactagaccagggcagtatttaggggaaggaggcagattggagcagttggctgccaacacctggcctcactcagggagaggggccttgggcctggatgatatctgggtgaggtacccacaccatctgctgcaacctctgtgtatccattatgggctcacgccattcacaggcatgaattgagcacctagtatgtgggaaaacaggggaaacagagatggcacagacatggtctccatccttcgggggctccagtctagttgggggagatcagagaagttccatttgccactctaggccaagctaggtaagcggcagagccatgaagcattgtgggagcttggaggagggagtgagcccttgcagtcagggagaaggagtcagcctggggagacttccagaaagtagccctttgaccctgaggaggtggggatcagtcgtgatgaaagtaatagccattcagtagccccttgtaattcaccctgagccaatgcctggaggcaggagaaagtactcaaggctctggtgcctggagccacaagacctggcggctttgtctaggcttcacccaagaaggatttatggagctccttcttggttctggtgttgctttgggcaccagggatgcaactgagtttaagacaggcatggcctccacctgcagggacttcagagcttgcctggggagagggtcacatggccagactgtgcagggtccccagtgcctatgagaggctttatcttaggacagtggagggccttgaggttttaaaagatagagccacatggacagaaagatcaatattgccctttatagtggctgctgcggttgtagctccgagactatattggagggggtgaggaaggacaagggggccagcaggtgggggacagcggcagacccctcccccaccccgatgctttggtccaaacaccacctctgagggctcccttgcttgggcttctcccaagattcccatccaccctcagaggacacagctactgcctcaactgggaggattcggaaagcttcagaaggtcagaaggcattggtagagggttccgggggaggctgggactacctccccccggagtgtttgaaaagccaggctggttcaggttagatactgaggtggggatgccagagctccatgctgaggaacagggtagagggtgtgggcttctagcacccaggggtctgcccccggcagtggggccgccagtagaaacgcagtcgcttctggtaggtgtccaggttgcgcttcaggcagaaggccacctccttgtcacaggcacacagctgctgctcacaccagcttcccttgtcagcagtccgtggcatctttgggttggcctctgccacctagtccgcagtgacagccgtagggccagtaggagaggatgggcattttcccagtcacttgcttgaccatcttgttcaggttcaggatcccgccctggattggaatcacaccagccatcaccaccagcccacacagcagtgcaagttccatgatcccagcacagagcagtggaggcagatgctggcagt

SEQ ID NO: 13829 - RNA, 2176 nt, Homo sapiens
  source 1..2176: mol_type = other RNA
gctgggattacaggcatgagccaccatgcctggcctctctgttcattattaaataccatgctgataattaagtctaaaatttagtctaagagtttccctttttcataatttctttaaaaacaaaggaggccagattaagtactatctatgtagatacttcttcagttctctggtttagcagtttaggtaatggctcatttaagttgaaatccactcaaatatctaagtcagaacactgtagacccaggcaagaatggcccttggaccgggccctgtgttttcaagtaacttcttgaccctcccgcagccatggccctctctacagagtaaggaatcagagagaccaaggagacagggccactggaatctacactctttgttctgaagcatgctgccagtcagtactcgagatcctgggttactcttcccaagtgggcccaagcctgctcacaggatctgcctggaccactttcctgtatacatcatcttgaagatgaacaacactgccagttttcacacccatccgctggaagggtgggagtggaggcgatgcttaggtgtgcaggctggaatgtccacatttgtgtgtgcaaggccccttacaatgtgggatggagccagagataggaaaagacagtattcagacatatggtgtgtgaaccccaaaaatctgagacaggtctcagataacttagaaagtttattttgccaaggttgaggacgtgcacccgtgacacagcctcagaaggtctgatgacatgtgcccaaggtggtggggcacagcttggttttgtacattttagggagacatgagacatcaatccatttgtgtaaggtgaatatcagttcagtccagaaaggtgggactactggaggcaaaggcggacaactgggagcgaggagggggcttccaggtcttaggcagataaaagacagatggttgtattcttttgagtttctgattagcctctccaaatgagacagtcagatatgcatttatctcagtgagcagaggggtgactttgaatagaatgggagccaggtttgccctaagcagttcccagcttgacttttcccttcagcttagtgatttgggggccccaagatttattttcctttaacagatgtatggacctacatttgtactcttgctctaggctctgaattattgggggttggtctgccctaaacctataccatccagtcacagtgcacaaatgaagaaccttatatatttgtaactcataaaatttcatgttttcttaagaggtttgattttcaaaaaaggtttatgtttatgttacaacttaagagtcttgtcaggagatagtatataaagcgggaatagctccaccatttcccaactgtagatagaccttgggcaagtccctgaaactccttatcctcatctataaaacgaagcacataatagcaactaacttaaagggtgattctgatgttaaatgaggtagtgcatggtgagaaaccccattcagtgcatggtaagcactcaatgagtgttggctattactgaccttgaggagttcagaaatctttcccttgtaaaggagcttaatccattgcgtccttactgctcatccatttacgttcctggtcagtgatgtgttgaaggaatgattttttaatagaggcttcaaattttctttgcttataactgtggcttagagatttggttttcctgatgtctactggtgtcatcagtggcttgctggcatctgatacttatctcttttcttttttggtagaatggatcttctaaccaaagacggagatttaatccacagtatcataacaacaggctaaatgggcctgccaagtcgcagggcagtgggaatgaagccgagccactgggaaagggcaacagccgccacgaacacagaagacagccgcacaacggcttccggcccaaaaacaaaggcggtgccaaaaatcaagaggcttccttggggatgaagacccccgaggccccggcccattctgaaaagccccggcgaaggcagcacgctgcagacacctcggaggccaggcccttccggggtagtgtcggtagggtttcacagtgcaatctctgccccacgagaatagaagtttccacagatgcagcagttctctcagtcccggctgtgacgttggtggcctgagctaggaggaaaaa

SEQ ID NO: 13830 - RNA, 3671 nt, Homo sapiens
  source 1..3671: mol_type = other RNA
gctgggattacaggcatgagccaccatgcctggcctgcttcaattttttgatgccactttgtaaacggcacttaattatggaaaataggaaaaagcaaaactaaaataaggaagaggatatatatataacttttcacaatctcttttctgattccctttagatgcccagtcaaccaggaccacacacagatttcattttatttgtagagtatatgaaaagatttaatagtctcatgcattttattttacgtatactgatttctacgttttgactgactatttaaataaacaaaacaagactcatttacaagggcatatactcttccttgtttggccagaagaaaatctatagctaaatctacttagaaaaacaatgctgctaaaactcttaacttcagattgtattaggctgagattttctaataacaaggttctttaaaattagaagggttcaatcccagcactttgggaggccgaggcaggtggatcacgaggtcaggagatcaagaccatcctggctaacacggtgaaaccctgtctctactaaaaatacaaaaaaatagccaggagtggtggtggacgcctgtagtcccagctattcgggaggcagggcaggagaatggcacgaacccgggaggcagagcttgcagtgagctgagatcatgccactacactccagcctgggcgacagagcaagactccgtctcaaaaaaaaaaaaaaaaaaaaaattagaagggttcctgaaaagtttgcaatggatgtggaaagtacttgagcttttactccaggaaatgctatacagattaaaattttaatccattagcagttaatgctgaaagcagaaatgctctcttaatcatttttccattcatcttttgaaatgttatttactcttgacaaaagtctgagtaccaagattcaggaaacacattccctacagaacaggtgtttgtttaatcccaagggatgatcttataggctgatttagtcagagacagcctggtgggagactccgatatagaacgttcatgctgtaattttaagtaccataataagtttgtagtagtataggctaggcttaaaactgcactcctcctgcctccccgcccccttccaaaaaaaagaaaaagtgaaaggaactctaaagagtgtcatatgcaggcacatctatataaaagctgggaaagaaattcatatccctgccattttcctttgtgtagttacccagtttaattcaactacctcaaaaaaaaaaaaaaagaaaaaataaaaggaaccctaaagagtgtcatatgtaggcacatctatataaaagctgggaaagaaattcatagccctgccattttcctttgtgtagttactcaatttaattcaactacttccacagaaatgtatgttagagaagagtatgctcagaaaggtattattgtgggtagctaacttcttgctttcaacaatggctgttctaaagtctggataacaaaaggggtggtggtctacttttcttcattaataatcaggtatctcattaaagccattcagaaaggcagagtaaattggggtggggagggtgagaagtgagtgtgaagaatattcaactatcttttgtaatatggtccccttaactaattctccttttttttttttgagactgagtctcgctctgtcacccaggctggagtacagtggcataatctcaactcaccgcaacctccgtctcctgggttcaagtgattctcctgtttcagcctcccgagtagcagggattacaggcgtgcactgctgcgcccggctaatttttttatttttagtagagacagggtttcactgtgttggcaaggctggtctcaaacttctgacttcagcagatccacccgcctcagcctcccaaagtgctgggattacaggtgtgagccaccatgcctgaccttgatattatcattttatccacagggtttgtcaaagggtatcctcattggcttgccagggcataagagagtttgactgagaaggcattagtgggctgtgtaatgactaactttgtaccactttctcaattagcaacatcagagatatcagagcaaatggtagatctttacagtgatgcagttaggagtttgttaactgccttttggaagtcagtgtaagaataagtagtgttgatgggttcagtacgagttgtttccttaactgttttagtcagccagccacagcaacacccagaaacacatgaattagggatctgttttaggtattcaggtatgggagtggctctactcaatgttcggcttagctgtttggtggcaaattgcagtgctccatttagagtggcatgatctctagagagccggctgggacttgtaagaggcttttgaaaaggtgggactccacaagaggccagagggggccattcaggaattggttccagtttggggacacaatgggaacaatgggagagtcttagacctatctctcgaagtatatggactggtgtgcttggatccaacagtttagcatgatacaaccaggaattaggatttaaaggtttccaagttgtggaatattttaaaaggcacttaacctgccaggcaagactctcaagaggcgataagttgggcaccatagagtcctcttcttcagaggaatcccactcttccccagaactctcatttaggtaactaatattttcttcttcctcactttctgattctgacaagtggtcaggagagggatttctaggacccatcagaataaaacacagtaaggaaccagaaaaaggtaataatctaagccagcagaacactgactaacactggcaaatagaaataagagatgaaaaatcctttcaccaagattaatttgtctttcagtccgttacacacataaagtatgcttgtggcccataccactgtgccgttcttcaagattatgttgtatattcttcacttacaaagaagacatctcagtttccaggaccagttcagtgtgtaaaagtattagtcacttaccactggcacaggtcagagtatctccttcaaatcctggctacccaagaatagaaggggtcctcatctaggcaagctgatttacttagcatagtcccaactggtagtgatactgtgaagagacactttttgtgctgttttgctggcagtgatattatatctacttgacaatcaaaagaagctcagtagttgtcttgcttgtccgctggtatagcaacttttgtgcaggggggaatgacgggatgagctgtcaagaacatctggtgtataaggatccgatgctttccataggtgatgcaaatgcccttggaaactggtgatttagctgttggattatctggaaaggtagccttaacctcgggtcgccccgctcagcggacccagcagcgtcgtctcccttctcagaggtggccgggcctccggaacgcgctacgaactttcctttgtcgccgtctctcgaagcggagccctcgtgtggggatcccccgcccttcggccacaagggaggttgttatcctcggcagatctcccgttctcactcttggaggatcgctttttctttctagcctcacgctcagccgcacgacccagccaggcctaacgccagcagcccttcccctccggtggcaaggccactccgctcagctcccgcgccgacgctactt

SEQ ID NO: 13831 - RNA, 3688 nt, Homo sapiens
  source 1..3688: mol_type = other RNA
gctgggattacaggcatgagccaccatgcctggcctgcttcaattttttgatgccactttgtaaacggcacttaattatggaaaataggaaaaagcaaaactaaaataaggaagaggatatatatataacttttcacaatctcttttctgattccctttagatgcccagtcaaccaggaccacacacagatttcattttatttgtagagtatatgaaaagatttaatagtctcatgcattttattttacgtatactgatttctacgttttgactgactatttaaataaacaaaacaagactcatttacaagggcatatactcttccttgtttggccagaagaaaatctatagctaaatctacttagaaaaacaatgctgctaaaactcttaacttcagattgtattaggctgagattttctaataacaaggttctttaaaattagaagggttcaatcccagcactttgggaggccgaggcaggtggatcacgaggtcaggagatcaagaccatcctggctaacacggtgaaaccctgtctctactaaaaatacaaaaaaatagccaggagtggtggtggacgcctgtagtcccagctattcgggaggcagggcaggagaatggcacgaacccgggaggcagagcttgcagtgagctgagatcatgccactacactccagcctgggcgacagagcaagactccgtctcaaaaaaaaaaaaaaaaaaaaaattagaagggttcctgaaaagtttgcaatggatgtggaaagtacttgagcttttactccaggaaatgctatacagattaaaattttaatccattagcagttaatgctgaaagcagaaatgctctcttaatcatttttccattcatcttttgaaatgttatttactcttgacaaaagtctgagtaccaagattcaggaaacacattccctacagaacaggtgtttgtttaatcccaagggatgatcttataggctgatttagtcagagacagcctggtgggagactccgatatagaacgttcatgctgtaattttaagtaccataataagtttgtagtagtataggctaggcttaaaactgcactcctcctgcctccccgcccccttccaaaaaaaagaaaaagtgaaaggaactctaaagagtgtcatatgcaggcacatctatataaaagctgggaaagaaattcatatccctgccattttcctttgtgtagttacccagtttaattcaactacctcaaaaaaaaaaaaaaagaaaaaataaaaggaaccctaaagagtgtcatatgtaggcacatctatataaaagctgggaaagaaattcatagccctgccattttcctttgtgtagttactcaatttaattcaactacttccacagaaatgtatgttagagaagagtatgctcagaaaggtattattgtgggtagctaacttcttgctttcaacaatggctgttctaaagtctggataacaaaaggggtggtggtctacttttcttcattaataatcaggtatctcattaaagccattcagaaaggcagagtaaattggggtggggagggtgagaagtgagtgtgaagaatattcaactatcttttgtaatatggtccccttaactaattctccttttttttttttgagactgagtctcgctctgtcacccaggctggagtacagtggcataatctcaactcaccgcaacctccgtctcctgggttcaagtgattctcctgtttcagcctcccgagtagcagggattacaggcgtgcactgctgcgcccggctaatttttttatttttagtagagacagggtttcactgtgttggcaaggctggtctcaaacttctgacttcagcagatccacccgcctcagcctcccaaagtgctgggattacaggtgtgagccaccatgcctgaccttgatattatcattttatccacagggtttgtcaaagggtatcctcattggcttgccagggcataagagagtttgactgagaaggcattagtgggctgtgtaatgactaactttgtaccactttctcaattagcaacatcagagatatcagagcaaatggtagatctttacagtgatgcagttaggagtttgttaactgccttttggaagtcagtgtaagaataagtagtgttgatgggttcagtacgagttgtttccttaactgttttagtcagccagccacagcaacacccagaaacacatgaattagggatctgttttaggtattcaggtatgggagtggctctactcaatgttcggcttagctgtttggtggcaaattgcagtgctccatttagagtggcatgatctctagagagccggctgggacttgtaagaggcttttgaaaaggtgggactccacaagaggccagagggggccattcaggaattggttccagtttggggacacaatgggaacaatgggagagtcttagacctatctctcgaagtatatggactggtgtgcttggatccaacagtttagcatgatacaaccaggaattaggatttaaaggtttccaagttgtggaatattttaaaaggcacttaacctgccaggcaagactctcaagaggcgataagttgggcaccatagagtcctcttcttcagaggaatcccactcttccccagaactctcatttaggtaactaatattttcttcttcctcactttctgattctgacaagtggtcaggagagggatttctaggacccatcagaataaaacacagtaaggaaccagaaaaaggtaataatctaagccagcagaacactgactaacactggcaaatagaaataagagatgaaaaatcctttcaccaagattaatttgtctttcagtccgttacacacataaagtatgcttgtggcccataccactgtgccgttcttcaagattatgttgtatattcttcacttacaaagaagacatctcagtttccaggaccagttcagtgtgtaaaagtattagtcacttaccactggcacaggtcagagtatctccttcaaatcctggctacccaagaatagaaggggtcctcatctaggcaagctgatttacttagcatagtcccaactggtagtgatactgtgaagagacactttttgtgctgttttgctggcagtgatattatatctacttgacaatcaaaagaagctcagtagttgtcttgcttgtccgctggtatagcaacttttgtgcaggggggaatgacgggatgagctgtcaagaacatctggtgtataaggatccgatgctttccataggtgatgcaaatgcccttggaaactggtgatttagctgttggattatctggaaaggtagccttaacctgtgaatgagaagactcgggtcgccccgctcagcggacccagcagcgtcgtctcccttctcagaggtggccgggcctccggaacgcgctacgaactttcctttgtcgccgtctctcgaagcggagccctcgtgtggggatcccccgcccttcggccacaagggaggttgttatcctcggcagatctcccgttctcactcttggaggatcgctttttctttctagcctcacgctcagccgcacgacccagccaggcctaacgccagcagcccttcccctccggtggcaaggccactccgctcagctcccgcgccgacgctacttcc

SEQ ID NO: 13832 - RNA, 3807 nt, Homo sapiens
  source 1..3807: mol_type = other RNA
gctgggattacaggcatgagccaccatgcctggcctgcttcaattttttgatgccactttgtaaacggcacttaattatggaaaataggaaaaagcaaaactaaaataaggaagaggatatatatataacttttcacaatctcttttctgattccctttagatgcccagtcaaccaggaccacacacagatttcattttatttgtagagtatatgaaaagatttaatagtctcatgcattttattttacgtatactgatttctacgttttgactgactatttaaataaacaaaacaagactcatttacaagggcatatactcttccttgtttggccagaagaaaatctatagctaaatctacttagaaaaacaatgctgctaaaactcttaacttcagattgtattaggctgagattttctaataacaaggttctttaaaattagaagggttcaatcccagcactttgggaggccgaggcaggtggatcacgaggtcaggagatcaagaccatcctggctaacacggtgaaaccctgtctctactaaaaatacaaaaaaatagccaggagtggtggtggacgcctgtagtcccagctattcgggaggcagggcaggagaatggcacgaacccgggaggcagagcttgcagtgagctgagatcatgccactacactccagcctgggcgacagagcaagactccgtctcaaaaaaaaaaaaaaaaaaaaaattagaagggttcctgaaaagtttgcaatggatgtggaaagtacttgagcttttactccaggaaatgctatacagattaaaattttaatccattagcagttaatgctgaaagcagaaatgctctcttaatcatttttccattcatcttttgaaatgttatttactcttgacaaaagtctgagtaccaagattcaggaaacacattccctacagaacaggtgtttgtttaatcccaagggatgatcttataggctgatttagtcagagacagcctggtgggagactccgatatagaacgttcatgctgtaattttaagtaccataataagtttgtagtagtataggctaggcttaaaactgcactcctcctgcctccccgcccccttccaaaaaaaagaaaaagtgaaaggaactctaaagagtgtcatatgcaggcacatctatataaaagctgggaaagaaattcatatccctgccattttcctttgtgtagttacccagtttaattcaactacctcaaaaaaaaaaaaaaagaaaaaataaaaggaaccctaaagagtgtcatatgtaggcacatctatataaaagctgggaaagaaattcatagccctgccattttcctttgtgtagttactcaatttaattcaactacttccacagaaatgtatgttagagaagagtatgctcagaaaggtattattgtgggtagctaacttcttgctttcaacaatggctgttctaaagtctggataacaaaaggggtggtggtctacttttcttcattaataatcaggtatctcattaaagccattcagaaaggcagagtaaattggggtggggagggtgagaagtgagtgtgaagaatattcaactatcttttgtaatatggtccccttaactaattctccttttttttttttgagactgagtctcgctctgtcacccaggctggagtacagtggcataatctcaactcaccgcaacctccgtctcctgggttcaagtgattctcctgtttcagcctcccgagtagcagggattacaggcgtgcactgctgcgcccggctaatttttttatttttagtagagacagggtttcactgtgttggcaaggctggtctcaaacttctgacttcagcagatccacccgcctcagcctcccaaagtgctgggattacaggtgtgagccaccatgcctgaccttgatattatcattttatccacagggtttgtcaaagggtatcctcattggcttgccagggcataagagagtttgactgagaaggcattagtgggctgtgtaatgactaactttgtaccactttctcaattagcaacatcagagatatcagagcaaatggtagatctttacagtgatgcagttaggagtttgttaactgccttttggaagtcagtgtaagaataagtagtgttgatgggttcagtacgagttgtttccttaactgttttagtcagccagccacagcaacacccagaaacacatgaattagggatctgttttaggtattcaggtatgggagtggctctactcaatgttcggcttagctgtttggtggcaaattgcagtgctccatttagagtggcatgatctctagagagccggctgggacttgtaagaggcttttgaaaaggtgggactccacaagaggccagagggggccattcaggaattggttccagtttggggacacaatgggaacaatgggagagtcttagacctatctctcgaagtatatggactggtgtgcttggatccaacagtttagcatgatacaaccaggaattaggatttaaaggtttccaagttgtggaatattttaaaaggcacttaacctgccaggcaagactctcaagaggcgataagttgggcaccatagagtcctcttcttcagaggaatcccactcttccccagaactctcatttaggtaactaatattttcttcttcctcactttctgattctgacaagtggtcaggagagggatttctaggacccatcagaataaaacacagtaaggaaccagaaaaaggtaataatctaagccagcagaacactgactaacactggcaaatagaaataagagatgaaaaatcctttcaccaagattaatttgtctttcagtccgttacacacataaagtatgcttgtggcccataccactgtgccgttcttcaagattatgttgtatattcttcacttacaaagaagacatctcagtttccaggaccagttcagtgtgtaaaagtattagtcacttaccactggcacaggtcagagtatctccttcaaatcctggctacccaagaatagaaggggtcctcatctaggcaagctgatttacttagcatagtcccaactggtagtgatactgtgaagagacactttttgtgctgttttgctggcagtgatattatatctacttgacaatcaaaagaagctcagtagttgtcttgcttgtccgctggtatagcaacttttgtgcaggggggaatgacgggatgagctgtcaagaacatctggtgtataaggatccgatgctttccataggtgatgcaaatgcccttggaaactggtgatttagctgttggattatctggaaaggtagccttaacctgtgaatgagaagacttcagaggtgcttgttggaattagttttagggggcctgtcctggtggtagagctgctagatgttaggactcttgctgggacctcagaagttgtgatcctatcaccaattctatataagctcgggtcgccccgctcagcggacccagcagcgtcgtctcccttctcagaggtggccgggcctccggaacgcgctacgaactttcctttgtcgccgtctctcgaagcggagccctcgtgtggggatcccccgcccttcggccacaagggaggttgttatcctcggcagatctcccgttctcactcttggaggatcgctttttctttctagcctcacgctcagccgcacgacccagccaggcctaacgccagcagcccttcccctccggtggcaaggccactccgctcagctcccgcgccgacgctacttcc

SEQ ID NO: 13833 - RNA, 3963 nt, Homo sapiens
  source 1..3963: mol_type = other RNA
gctgggattacaggcatgagccaccatgcctggcctgcttcaattttttgatgccactttgtaaacggcacttaattatggaaaataggaaaaagcaaaactaaaataaggaagaggatatatatataacttttcacaatctcttttctgattccctttagatgcccagtcaaccaggaccacacacagatttcattttatttgtagagtatatgaaaagatttaatagtctcatgcattttattttacgtatactgatttctacgttttgactgactatttaaataaacaaaacaagactcatttacaagggcatatactcttccttgtttggccagaagaaaatctatagctaaatctacttagaaaaacaatgctgctaaaactcttaacttcagattgtattaggctgagattttctaataacaaggttctttaaaattagaagggttcaatcccagcactttgggaggccgaggcaggtggatcacgaggtcaggagatcaagaccatcctggctaacacggtgaaaccctgtctctactaaaaatacaaaaaaatagccaggagtggtggtggacgcctgtagtcccagctattcgggaggcagggcaggagaatggcacgaacccgggaggcagagcttgcagtgagctgagatcatgccactacactccagcctgggcgacagagcaagactccgtctcaaaaaaaaaaaaaaaaaaaaaattagaagggttcctgaaaagtttgcaatggatgtggaaagtacttgagcttttactccaggaaatgctatacagattaaaattttaatccattagcagttaatgctgaaagcagaaatgctctcttaatcatttttccattcatcttttgaaatgttatttactcttgacaaaagtctgagtaccaagattcaggaaacacattccctacagaacaggtgtttgtttaatcccaagggatgatcttataggctgatttagtcagagacagcctggtgggagactccgatatagaacgttcatgctgtaattttaagtaccataataagtttgtagtagtataggctaggcttaaaactgcactcctcctgcctccccgcccccttccaaaaaaaagaaaaagtgaaaggaactctaaagagtgtcatatgcaggcacatctatataaaagctgggaaagaaattcatatccctgccattttcctttgtgtagttacccagtttaattcaactacctcaaaaaaaaaaaaaaagaaaaaataaaaggaaccctaaagagtgtcatatgtaggcacatctatataaaagctgggaaagaaattcatagccctgccattttcctttgtgtagttactcaatttaattcaactacttccacagaaatgtatgttagagaagagtatgctcagaaaggtattattgtgggtagctaacttcttgctttcaacaatggctgttctaaagtctggataacaaaaggggtggtggtctacttttcttcattaataatcaggtatctcattaaagccattcagaaaggcagagtaaattggggtggggagggtgagaagtgagtgtgaagaatattcaactatcttttgtaatatggtccccttaactaattctccttttttttttttgagactgagtctcgctctgtcacccaggctggagtacagtggcataatctcaactcaccgcaacctccgtctcctgggttcaagtgattctcctgtttcagcctcccgagtagcagggattacaggcgtgcactgctgcgcccggctaatttttttatttttagtagagacagggtttcactgtgttggcaaggctggtctcaaacttctgacttcagcagatccacccgcctcagcctcccaaagtgctgggattacaggtgtgagccaccatgcctgaccttgatattatcattttatccacagggtttgtcaaagggtatcctcattggcttgccagggcataagagagtttgactgagaaggcattagtgggctgtgtaatgactaactttgtaccactttctcaattagcaacatcagagatatcagagcaaatggtagatctttacagtgatgcagttaggagtttgttaactgccttttggaagtcagtgtaagaataagtagtgttgatgggttcagtacgagttgtttccttaactgttttagtcagccagccacagcaacacccagaaacacatgaattagggatctgttttaggtattcaggtatgggagtggctctactcaatgttcggcttagctgtttggtggcaaattgcagtgctccatttagagtggcatgatctctagagagccggctgggacttgtaagaggcttttgaaaaggtgggactccacaagaggccagagggggccattcaggaattggttccagtttggggacacaatgggaacaatgggagagtcttagacctatctctcgaagtatatggactggtgtgcttggatccaacagtttagcatgatacaaccaggaattaggatttaaaggtttccaagttgtggaatattttaaaaggcacttaacctgccaggcaagactctcaagaggcgataagttgggcaccatagagtcctcttcttcagaggaatcccactcttccccagaactctcatttaggtaactaatattttcttcttcctcactttctgattctgacaagtggtcaggagagggatttctaggacccatcagaataaaacacagtaaggaaccagaaaaaggtaataatctaagccagcagaacactgactaacactggcaaatagaaataagagatgaaaaatcctttcaccaagattaatttgtctttcagtccgttacacacataaagtatgcttgtggcccataccactgtgccgttcttcaagattatgttgtatattcttcacttacaaagaagacatctcagtttccaggaccagttcagtgtgtaaaagtattagtcacttaccactggcacaggtcagagtatctccttcaaatcctggctacccaagaatagaaggggtcctcatctaggcaagctgatttacttagcatagtcccaactggtagtgatactgtgaagagacactttttgtgctgttttgctggcagtgatattatatctacttgacaatcaaaagaagctcagtagttgtcttgcttgtccgctggtatagcaacttttgtgcaggggggaatgacgggatgagctgtcaagaacatctggtgtataaggatccgatgctttccataggtgatgcaaatgcccttggaaactggtgatttagctgttggattatctggaaaggtagccttaacctgtgaatgagaagacttcagaggtgcttgttggaattagttttagggggcctgtcctggtggtagagctgctagatgttaggactcttgctgggacctcagaagttgtgatcctatcaccaattctatataagttcttcggagggcaggtaattcaaaaggagaaagatgtacaggtggctttagtaatgttctatttcttcagctggcagtaggttactgaggtgtaggagagggaaaaacggcttccctccatcctcctaggttctttggctgggttacaaattaacctcgggtcgccccgctcagcggacccagcagcgtcgtctcccttctcagaggtggccgggcctccggaacgcgctacgaactttcctttgtcgccgtctctcgaagcggagccctcgtgtggggatcccccgcccttcggccacaagggaggttgttatcctcggcagatctcccgttctcactcttggaggatcgctttttctttctagcctcacgctcagccgcacgacccagccaggcctaacgccagcagcccttcccctccggtggcaaggccactccgctcagctcccgcgccgacgctacttcc

SEQ ID NO: 13834 - RNA, 3724 nt, Homo sapiens
  source 1..3724: mol_type = other RNA
gctgggattacaggcatgagccaccatgcctggcctgcttcaattttttgatgccactttgtaaacggcacttaattatggaaaataggaaaaagcaaaactaaaataaggaagaggatatatatataacttttcacaatctcttttctgattccctttagatgcccagtcaaccaggaccacacacagatttcattttatttgtagagtatatgaaaagatttaatagtctcatgcattttattttacgtatactgatttctacgttttgactgactatttaaataaacaaaacaagactcatttacaagggcatatactcttccttgtttggccagaagaaaatctatagctaaatctacttagaaaaacaatgctgctaaaactcttaacttcagattgtattaggctgagattttctaataacaaggttctttaaaattagaagggttcaatcccagcactttgggaggccgaggcaggtggatcacgaggtcaggagatcaagaccatcctggctaacacggtgaaaccctgtctctactaaaaatacaaaaaaatagccaggagtggtggtggacgcctgtagtcccagctattcgggaggcagggcaggagaatggcacgaacccgggaggcagagcttgcagtgagctgagatcatgccactacactccagcctgggcgacagagcaagactccgtctcaaaaaaaaaaaaaaaaaaaaaattagaagggttcctgaaaagtttgcaatggatgtggaaagtacttgagcttttactccaggaaatgctatacagattaaaattttaatccattagcagttaatgctgaaagcagaaatgctctcttaatcatttttccattcatcttttgaaatgttatttactcttgacaaaagtctgagtaccaagattcaggaaacacattccctacagaacaggtgtttgtttaatcccaagggatgatcttataggctgatttagtcagagacagcctggtgggagactccgatatagaacgttcatgctgtaattttaagtaccataataagtttgtagtagtataggctaggcttaaaactgcactcctcctgcctccccgcccccttccaaaaaaaagaaaaagtgaaaggaactctaaagagtgtcatatgcaggcacatctatataaaagctgggaaagaaattcatatccctgccattttcctttgtgtagttacccagtttaattcaactacctcaaaaaaaaaaaaaaagaaaaaataaaaggaaccctaaagagtgtcatatgtaggcacatctatataaaagctgggaaagaaattcatagccctgccattttcctttgtgtagttactcaatttaattcaactacttccacagaaatgtatgttagagaagagtatgctcagaaaggtattattgtgggtagctaacttcttgctttcaacaatggctgttctaaagtctggataacaaaaggggtggtggtctacttttcttcattaataatcaggtatctcattaaagccattcagaaaggcagagtaaattggggtggggagggtgagaagtgagtgtgaagaatattcaactatcttttgtaatatggtccccttaactaattctccttttttttttttgagactgagtctcgctctgtcacccaggctggagtacagtggcataatctcaactcaccgcaacctccgtctcctgggttcaagtgattctcctgtttcagcctcccgagtagcagggattacaggcgtgcactgctgcgcccggctaatttttttatttttagtagagacagggtttcactgtgttggcaaggctggtctcaaacttctgacttcagcagatccacccgcctcagcctcccaaagtgctgggattacaggtgtgagccaccatgcctgaccttgatattatcattttatccacagggtttgtcaaagggtatcctcattggcttgccagggcataagagagtttgactgagaaggcattagtgggctgtgtaatgactaactttgtaccactttctcaattagcaacatcagagatatcagagcaaatggtagatctttacagtgatgcagttaggagtttgttaactgccttttggaagtcagtgtaagaataagtagtgttgatgggttcagtacgagttgtttccttaactgttttagtcagccagccacagcaacacccagaaacacatgaattagggatctgttttaggtattcaggtatgggagtggctctactcaatgttcggcttagctgtttggtggcaaattgcagtgctccatttagagtggcatgatctctagagagccggctgggacttgtaagaggcttttgaaaaggtgggactccacaagaggccagagggggccattcaggaattggttccagtttggggacacaatgggaacaatgggagagtcttagacctatctctcgaagtatatggactggtgtgcttggatccaacagtttagcatgatacaaccaggaattaggatttaaaggtttccaagttgtggaatattttaaaaggcacttaacctgccaggcaagactctcaagaggcgataagttgggcaccatagagtcctcttcttcagaggaatcccactcttccccagaactctcatttaggtaactaatattttcttcttcctcactttctgattctgacaagtggtcaggagagggatttctaggacccatcagaataaaacacagtaaggaaccagaaaaaggtaataatctaagccagcagaacactgactaacactggcaaatagaaataagagatgaaaaatcctttcaccaagattaatttgtctttcagtccgttacacacataaagtatgcttgtggcccataccactgtgccgttcttcaagattatgttgtatattcttcacttacaaagaagacatctcagtttccaggaccagttcagtgtgtaaaagtattagtcacttaccactggcacaggtcagagtatctccttcaaatcctggctacccaagaatagaaggggtcctcatctaggcaagctgatttacttagcatagtcccaactggtagtgatactgtgaagagacactttttgtgctgttttgctggcagtgatattatatctacttgacaatcaaaagaagctcagtagttgtcttgcttgtccgctggtatagcaacttttgtgcaggggggaatgacgggatgagctgtcaagaacatctggtgtataaggatccgatgctttccataggtgatgcaaatgcccttggaaactggtgatttagctgttggattatctggaaaggtagccttaacctgtgaatgagaagacttcagaggtgcttgttggaattagttttagggggcctgtcctggtggtagagctgggacccagcagcgtcgtctcccttctcagaggtggccgggcctccggaacgcgctacgaactttcctttgtcgccgtctctcgaagcggagccctcgtgtggggatcccccgcccttcggccacaagggaggttgttatcctcggcagatctcccgttctcactcttggaggatcgctttttctttctagcctcacgctcagccgcacgacccagccaggcctaacgccagcagcccttcccctccggtggcaaggccactccgctcagctcccgcgccgacgctacttcc

SEQ ID NO: 13835 - RNA, 3792 nt, Homo sapiens
  source 1..3792: mol_type = other RNA
gctgggattacaggcatgagccaccatgcctggcctgcttcaattttttgatgccactttgtaaacggcacttaattatggaaaataggaaaaagcaaaactaaaataaggaagaggatatatatataacttttcacaatctcttttctgattccctttagatgcccagtcaaccaggaccacacacagatttcattttatttgtagagtatatgaaaagatttaatagtctcatgcattttattttacgtatactgatttctacgttttgactgactatttaaataaacaaaacaagactcatttacaagggcatatactcttccttgtttggccagaagaaaatctatagctaaatctacttagaaaaacaatgctgctaaaactcttaacttcagattgtattaggctgagattttctaataacaaggttctttaaaattagaagggttcaatcccagcactttgggaggccgaggcaggtggatcacgaggtcaggagatcaagaccatcctggctaacacggtgaaaccctgtctctactaaaaatacaaaaaaatagccaggagtggtggtggacgcctgtagtcccagctattcgggaggcagggcaggagaatggcacgaacccgggaggcagagcttgcagtgagctgagatcatgccactacactccagcctgggcgacagagcaagactccgtctcaaaaaaaaaaaaaaaaaaaaaattagaagggttcctgaaaagtttgcaatggatgtggaaagtacttgagcttttactccaggaaatgctatacagattaaaattttaatccattagcagttaatgctgaaagcagaaatgctctcttaatcatttttccattcatcttttgaaatgttatttactcttgacaaaagtctgagtaccaagattcaggaaacacattccctacagaacaggtgtttgtttaatcccaagggatgatcttataggctgatttagtcagagacagcctggtgggagactccgatatagaacgttcatgctgtaattttaagtaccataataagtttgtagtagtataggctaggcttaaaactgcactcctcctgcctccccgcccccttccaaaaaaaagaaaaagtgaaaggaactctaaagagtgtcatatgcaggcacatctatataaaagctgggaaagaaattcatatccctgccattttcctttgtgtagttacccagtttaattcaactacctcaaaaaaaaaaaaaaagaaaaaataaaaggaaccctaaagagtgtcatatgtaggcacatctatataaaagctgggaaagaaattcatagccctgccattttcctttgtgtagttactcaatttaattcaactacttccacagaaatgtatgttagagaagagtatgctcagaaaggtattattgtgggtagctaacttcttgctttcaacaatggctgttctaaagtctggataacaaaaggggtggtggtctacttttcttcattaataatcaggtatctcattaaagccattcagaaaggcagagtaaattggggtggggagggtgagaagtgagtgtgaagaatattcaactatcttttgtaatatggtccccttaactaattctccttttttttttttgagactgagtctcgctctgtcacccaggctggagtacagtggcataatctcaactcaccgcaacctccgtctcctgggttcaagtgattctcctgtttcagcctcccgagtagcagggattacaggcgtgcactgctgcgcccggctaatttttttatttttagtagagacagggtttcactgtgttggcaaggctggtctcaaacttctgacttcagcagatccacccgcctcagcctcccaaagtgctgggattacaggtgtgagccaccatgcctgaccttgatattatcattttatccacagggtttgtcaaagggtatcctcattggcttgccagggcataagagagtttgactgagaaggcattagtgggctgtgtaatgactaactttgtaccactttctcaattagcaacatcagagatatcagagcaaatggtagatctttacagtgatgcagttaggagtttgttaactgccttttggaagtcagtgtaagaataagtagtgttgatgggttcagtacgagttgtttccttaactgttttagtcagccagccacagcaacacccagaaacacatgaattagggatctgttttaggtattcaggtatgggagtggctctactcaatgttcggcttagctgtttggtggcaaattgcagtgctccatttagagtggcatgatctctagagagccggctgggacttgtaagaggcttttgaaaaggtgggactccacaagaggccagagggggccattcaggaattggttccagtttggggacacaatgggaacaatgggagagtcttagacctatctctcgaagtatatggactggtgtgcttggatccaacagtttagcatgatacaaccaggaattaggatttaaaggtttccaagttgtggaatattttaaaaggcacttaacctgccaggcaagactctcaagaggcgataagttgggcaccatagagtcctcttcttcagaggaatcccactcttccccagaactctcatttaggtaactaatattttcttcttcctcactttctgattctgacaagtggtcaggagagggatttctaggacccatcagaataaaacacagtaaggaaccagaaaaaggtaataatctaagccagcagaacactgactaacactggcaaatagaaataagagatgaaaaatcctttcaccaagattaatttgtctttcagtccgttacacacataaagtatgcttgtggcccataccactgtgccgttcttcaagattatgttgtatattcttcacttacaaagaagacatctcagtttccaggaccagttcagtgtgtaaaagtattagtcacttaccactggcacaggtcagagtatctccttcaaatcctggctacccaagaatagaaggggtcctcatctaggcaagctgatttacttagcatagtcccaactggtagtgatactgtgaagagacactttttgtgctgttttgctggcagtgatattatatctacttgacaatcaaaagaagctcagtagttgtcttgcttgtccgctggtatagcaacttttgtgcaggggggaatgacgggatgagctgtcaagaacatctggtgtataaggatccgatgctttccataggtgatgcaaatgcccttggaaactggtgatttagctgttggattatctggaaaggtagccttaaccttcagaggtgcttgttggaattagttttagggggcctgtcctggtggtagagctgctagatgttaggactcttgctgggacctcagaagttgtgatcctatcaccaattctatataagctcgggtcgccccgctcagcggacccagcagcgtcgtctcccttctcagaggtggccgggcctccggaacgcgctacgaactttcctttgtcgccgtctctcgaagcggagccctcgtgtggggatcccccgcccttcggccacaagggaggttgttatcctcggcagatctcccgttctcactcttggaggatcgctttttctttctagcctcacgctcagccgcacgacccagccaggcctaacgccagcagcccttcccctccggtggcaaggccactccgctcagctcccgcgccgacgctacttcc

SEQ ID NO: 13836 - RNA, 3829 nt, Homo sapiens
  source 1..3829: mol_type = other RNA
gctgggattacaggcatgagccaccatgcctggcctgcttcaattttttgatgccactttgtaaacggcacttaattatggaaaataggaaaaagcaaaactaaaataaggaagaggatatatatataacttttcacaatctcttttctgattccctttagatgcccagtcaaccaggaccacacacagatttcattttatttgtagagtatatgaaaagatttaatagtctcatgcattttattttacgtatactgatttctacgttttgactgactatttaaataaacaaaacaagactcatttacaagggcatatactcttccttgtttggccagaagaaaatctatagctaaatctacttagaaaaacaatgctgctaaaactcttaacttcagattgtattaggctgagattttctaataacaaggttctttaaaattagaagggttcaatcccagcactttgggaggccgaggcaggtggatcacgaggtcaggagatcaagaccatcctggctaacacggtgaaaccctgtctctactaaaaatacaaaaaaatagccaggagtggtggtggacgcctgtagtcccagctattcgggaggcagggcaggagaatggcacgaacccgggaggcagagcttgcagtgagctgagatcatgccactacactccagcctgggcgacagagcaagactccgtctcaaaaaaaaaaaaaaaaaaaaaattagaagggttcctgaaaagtttgcaatggatgtggaaagtacttgagcttttactccaggaaatgctatacagattaaaattttaatccattagcagttaatgctgaaagcagaaatgctctcttaatcatttttccattcatcttttgaaatgttatttactcttgacaaaagtctgagtaccaagattcaggaaacacattccctacagaacaggtgtttgtttaatcccaagggatgatcttataggctgatttagtcagagacagcctggtgggagactccgatatagaacgttcatgctgtaattttaagtaccataataagtttgtagtagtataggctaggcttaaaactgcactcctcctgcctccccgcccccttccaaaaaaaagaaaaagtgaaaggaactctaaagagtgtcatatgcaggcacatctatataaaagctgggaaagaaattcatatccctgccattttcctttgtgtagttacccagtttaattcaactacctcaaaaaaaaaaaaaaagaaaaaataaaaggaaccctaaagagtgtcatatgtaggcacatctatataaaagctgggaaagaaattcatagccctgccattttcctttgtgtagttactcaatttaattcaactacttccacagaaatgtatgttagagaagagtatgctcagaaaggtattattgtgggtagctaacttcttgctttcaacaatggctgttctaaagtctggataacaaaaggggtggtggtctacttttcttcattaataatcaggtatctcattaaagccattcagaaaggcagagtaaattggggtggggagggtgagaagtgagtgtgaagaatattcaactatcttttgtaatatggtccccttaactaattctccttttttttttttgagactgagtctcgctctgtcacccaggctggagtacagtggcataatctcaactcaccgcaacctccgtctcctgggttcaagtgattctcctgtttcagcctcccgagtagcagggattacaggcgtgcactgctgcgcccggctaatttttttatttttagtagagacagggtttcactgtgttggcaaggctggtctcaaacttctgacttcagcagatccacccgcctcagcctcccaaagtgctgggattacaggtgtgagccaccatgcctgaccttgatattatcattttatccacagggtttgtcaaagggtatcctcattggcttgccagggcataagagagtttgactgagaaggcattagtgggctgtgtaatgactaactttgtaccactttctcaattagcaacatcagagatatcagagcaaatggtagatctttacagtgatgcagttaggagtttgttaactgccttttggaagtcagtgtaagaataagtagtgttgatgggttcagtacgagttgtttccttaactgttttagtcagccagccacagcaacacccagaaacacatgaattagggatctgttttaggtattcaggtatgggagtggctctactcaatgttcggcttagctgtttggtggcaaattgcagtgctccatttagagtggcatgatctctagagagccggctgggacttgtaagaggcttttgaaaaggtgggactccacaagaggccagagggggccattcaggaattggttccagtttggggacacaatgggaacaatgggagagtcttagacctatctctcgaagtatatggactggtgtgcttggatccaacagtttagcatgatacaaccaggaattaggatttaaaggtttccaagttgtggaatattttaaaaggcacttaacctgccaggcaagactctcaagaggcgataagttgggcaccatagagtcctcttcttcagaggaatcccactcttccccagaactctcatttaggtaactaatattttcttcttcctcactttctgattctgacaagtggtcaggagagggatttctaggacccatcagaataaaacacagtaaggaaccagaaaaaggtaataatctaagccagcagaacactgactaacactggcaaatagaaataagagatgaaaaatcctttcaccaagattaatttgtctttcagtccgttacacacataaagtatgcttgtggcccataccactgtgccgttcttcaagattatgttgtatattcttcacttacaaagaagacatctcagtttccaggaccagttcagtgtgtaaaagtattagtcacttaccactggcacaggtcagagtatctccttcaaatcctggctacccaagaatagaaggggtcctcatctaggcaagctgatttacttagcatagtcccaactggtagtgatactgtgaagagacactttttgtgctgttttgctggcagtgatattatatctacttgacaatcaaaagaagctcagtagttgtcttgcttgtccgctggtatagcaacttttgtgcaggggggaatgacgggatgagctgtcaagaacatctggtgtataaggatccgatgctttccataggtgatgcaaatgcccttggaaactggtgatttagctgttggattatctggaaaggtagccttaacttcttcggagggcaggtaattcaaaaggagaaagatgtacaggtggctttagtaatgttctatttcttcagctggcagtaggttactgaggtgtaggagagggaaaaacggcttccctccatcctcctaggttctttggctgggttacaaattaacctcgggtcgccccgctcagcggacccagcagcgtcgtctcccttctcagaggtggccgggcctccggaacgcgctacgaactttcctttgtcgccgtctctcgaagcggagccctcgtgtggggatcccccgcccttcggccacaagggaggttgttatcctcggcagatctcccgttctcactcttggaggatcgctttttctttctagcctcacgctcagccgcacgacccagccaggcctaacgccagcagcccttcccctccggtggcaaggccactccgctcagctcccgcgccgacgctacttcc

SEQ ID NO: 13837 - RNA, 3640 nt, Homo sapiens
  source 1..3640: mol_type = other RNA
gctgggattacaggcatgagccaccatgcctggcctgtaaataaagttttactggaacacagccatgctcttctgtttacatcttgtctatggctgctttagtgctacaatggcagagttgggtagttgggacagacaccatgtctgtctgttggtacagacaacacaaactccaaaatatgtactctgtgggtctttactgaaaactttgccgacccttggtctagacagatagtcagatgagctaacagttggctaaaggtcctcaactcacaatgccaagagaaggactgagttggctttagttgttgtcatgcactgtgtaatttaaaaaatcttacaggccagtacaactaaaactcctatttaccttactttggagcaacaatatggaaagtaaaactaggtctgaatatattttatatgttacctggacttctaaaacattgttgattgcttaaatgtgcataagtcaatgtcatttctcaaaacgtttaatagatgcaactgttggcggctgctaaagtactggtgttatgcttgtgcctgtgtgaaattctacagtgctgaaaatctcatgcactctagctatgaatgcaggtctacttgaagcaaaactcttcaatctaattgttttctcaatctttgtaaaccagttttaagagtcaccagaaatctgtagtttaaggcaccagatacatttcttggctgagccttgtaggaccaatatgctggaccaattcggtaaaatacaccataaattatgactgctttatctgaatgcatgggacacttgctacgatggcgggaattattaccaggagtttaggagccagacatgggttctgtatttttcatacattggtgatcaattcaaatctctttcctttgcagccaggtttggtcagtctggccaggagtgcagattatgacaaagaacaaagctaaaagacctgagccattaaggttacagtctcaataccaccgagttaaacaacctatttaaatgcaagactattgattggaatgatattggacagacatgtcagaagtgatctgaaggctttgaaatgtcattaagggtgggacttattgttggatgttggctgcaacgaaggctacttcttttcttctcctttaaatattaggtagatcataaataacagatattattatggattctacctgcaaatgtgtcttagcagatatgtgatgaattggagtggaaaagccattcaggaaacaggaggacttgggcttcctcttgaagctcaggtttgaccactgggttgttttctatgtctacaggtttaaatggctgaaattcagttctctaatcacaactctccttttatctagaagaatttacaaagcttgaggtaatgactttgggaagaaatgatgtgtagtgaaactatcactaagaatttaaatgtgattttttagacttatatggagaataagacatataaatccacttgataaattataagatctataaaaaagacataggatattaaatttttcttcagtttcaagtatgatagaatcatacagctgaagaaaacatcaccattctagatttttattaaaaaataaacaaacattagtcctactttttgtctctaacgcttcatgaatttatgtgtcagccttgtgcaggggctgtgctaatctctgcattgttcctattttagtacatgggctactgaaacaagcagagtcctacttcttaaacttcctcttccttacacgtaaaaagcccaccagtcaaggtcttttaattttggtgtacactatcactgaatgccatttataaattctaattttaaagagacccttaattttcaaaggaggactttgatagcattagttttcagaaaagatgacttgcaattctaacttagtacttgaaaggtgagatttttatagggaggcttataaaaggtgtcttagaaaaaaaatgagcgctctcaaacctttcttttgggagtgaggttgtggggctgaagtgactttttaaagtgaagcaactgacactacccgtgggagaagccacctatgcgacctgtggccaaaccgcaaatgtatgtttctgtgcaacattcctgctagagcagccgggctctgagtaaggtgtagctggctagataatcactagggagaggtccagggtgtggggaacactccaaatcacattccatggaaatattagactgtcagagcttaggaagtccccgattgtccatagacgctgaggtgggggaaaggactgaaatgaatgctagcacatgttagcttataaaagagctgctgacacaaattgaacatgtgcaattttttaaaaaggtggtatcgaataacaggccaacagccatccttctcagcatttagacctctttcttctctccactttggctctttgttgagtcacttccatcaggcaaagttccataggataagctatgtgaatctggttgtattttgtccaacatttgtttcccaggaatatttccaaaatcaatataagactgttgcagatgttccttttctcgatttcttgtgaccaaaaatacaccaaggaatgacagaaaacacccaaaaagatatataaatacagtgagaaaaggagcaccaaggaattcctgataaaatatgatacctgcaatgatggcactgattgtaaagaaaatatgattaactggcaccactgttgtcgtattgtagagtttcgtggcttgattcaggaacttgacttggaaaacacaagatgctatcatgatgataaacatgatatagaaaatggggtaagttagttgcattttatccatcacagaaaaagtgatcatgcctgagacggcctttactgaaataacagtcaatgaggctagaattgccaccagggttagcagaatcaccatatgcttcattccttttcttttatagaaatacaggagaatgcagaaaattaatatttctaaaatcacatagatcaggaactgccatccgacaaggtaatactgtactgttcttgctgagattgcctgagttatatttggagcaaagttcaccagtaaatatgttcctgcaaatgccagtgtcgtaccgagtaagtctgaggctctcaaattgtctttcagaaatgtaacagaaataatggcactacctgtaacagacacacagcctaacggagcgatcagagtaatgggagcaaatccataggctgcaaagttccccgtctctcccacggccatcagcaggacaccaccccaccacagcacactcttgaagtatggccttgggtgctcttgttgtgccagctgaaggtgagaatatttctgaatatttagagaaatactgatcaccaagtttcctaaaatagccagcaaaactccaaaaaggtgaatctggttcctgcggtaccagtcgcccgagagggagccgttgccggcgcctggtgccccgtacgtgaaattcagtgacagctcgtccagggcggccgaggcggagtccccggggcccgcgggcgccaccgctgccatgaggtctcgctcccggcgctcgggctccggctcgggctgcggccgcctccccgccctgttgcaccgcgaggaggccgcgccgcagccacttcctgctc

SEQ ID NO: 13838 - RNA, 3926 nt, Homo sapiens
  source 1..3926: mol_type = other RNA
gctgggattacaggcatgagccaccatgcctggcctgtaaataaagttttactggaacacagccatgctcttctgtttacatcttgtctatggctgctttagtgctacaatggcagagttgggtagttgggacagacaccatgtctgtctgttggtacagacaacacaaactccaaaatatgtactctgtgggtctttactgaaaactttgccgacccttggtctagacagatagtcagatgagctaacagttggctaaaggtcctcaactcacaatgccaagagaaggactgagttggctttagttgttgtcatgcactgtgtaatttaaaaaatcttacaggccagtacaactaaaactcctatttaccttactttggagcaacaatatggaaagtaaaactaggtctgaatatattttatatgttacctggacttctaaaacattgttgattgcttaaatgtgcataagtcaatgtcatttctcaaaacgtttaatagatgcaactgttggcggctgctaaagtactggtgttatgcttgtgcctgtgtgaaattctacagtgctgaaaatctcatgcactctagctatgaatgcaggtctacttgaagcaaaactcttcaatctaattgttttctcaatctttgtaaaccagttttaagagtcaccagaaatctgtagtttaaggcaccagatacatttcttggctgagccttgtaggaccaatatgctggaccaattcggtaaaatacaccataaattatgactgctttatctgaatgcatgggacacttgctacgatggcgggaattattaccaggagtttaggagccagacatgggttctgtatttttcatacattggtgatcaattcaaatctctttcctttgcagccaggtttggtcagtctggccaggagtgcagattatgacaaagaacaaagctaaaagacctgagccattaaggttacagtctcaataccaccgagttaaacaacctatttaaatgcaagactattgattggaatgatattggacagacatgtcagaagtgatctgaaggctttgaaatgtcattaagggtgggacttattgttggatgttggctgcaacgaaggctacttcttttcttctcctttaaatattaggtagatcataaataacagatattattatggattctacctgcaaatgtgtcttagcagatatgtgatgaattggagtggaaaagccattcaggaaacaggaggacttgggcttcctcttgaagctcaggtttgaccactgggttgttttctatgtctacaggtttaaatggctgaaattcagttctctaatcacaactctccttttatctagaagaatttacaaagcttgaggtaatgactttgggaagaaatgatgtgtagtgaaactatcactaagaatttaaatgtgattttttagacttatatggagaataagacatataaatccacttgataaattataagatctataaaaaagacataggatattaaatttttcttcagtttcaagtatgatagaatcatacagctgaagaaaacatcaccattctagatttttattaaaaaataaacaaacattagtcctactttttgtctctaacgcttcatgaatttatgtgtcagccttgtgcaggggctgtgctaatctctgcattgttcctattttagtacatgggctactgaaacaagcagagtcctacttcttaaacttcctcttccttacacgtaaaaagcccaccagtcaaggtcttttaattttggtgtacactatcactgaatgccatttataaattctaattttaaagagacccttaattttcaaaggaggactttgatagcattagttttcagaaaagatgacttgcaattctaacttagtacttgaaaggtgagatttttatagggaggcttataaaaggtgtcttagaaaaaaaatgagcgctctcaaacctttcttttgggagtgaggttgtggggctgaagtgactttttaaagtgaagcaactgacactacccgtgggagaagccacctatgcgacctgtggccaaaccgcaaatgtatgtttctgtgcaacattcctgctagagcagccgggctctgagtaaggtgtagctggctagataatcactagggagaggtccagggtgtggggaacactccaaatcacattccatggaaatattagactgtcagagcttaggaagtccccgattgtccatagacgctgaggtgggggaaaggactgaaatgaatgctagcacatgttagcttataaaagagctgctgacacaaattgaacatgtgcaattttttaaaaaggtggtatcgaataacaggccaacagccatccttctcagcatttagacctctttcttctctccactttggctctttgttgagtcacttccatcaggcaaagttccataggataagctatgtgaatctggttgtattttgtccaacatttgtttcccaggaatatttccaaaatcaatataagactgttgcagatgttccttttctcgatttcttgtgaccaaaaatacaccaaggaatgacagaaaacacccaaaaagatatataaatacagtgagaaaaggagcaccaaggaattcctgataaaatatgatacctgcaatgatggcactgattgtaaagaaaatatgattaactggcaccactgttgtcgtattgtagagtttcgtggcttgattcaggaacttgacttggaaaacacaagatgctatcatgatgataaacatgatatagaaaatggggtaagttagttgcattttatccatcacagaaaaagtgatcatgcctgagacggcctttactgaaataacagtcaatgaggctagaattgccaccagggttagcagaatcaccatatgcttcattccttttcttttatagaaatacaggagaatgcagaaaattaatatttctaaaatcacatagatcaggaactgccatccgacaaggtaatactgtactgttcttgctgagattgcctgagttatatttggagcaaagttcaccagtaaatatgttcctgcaaatgccagtgtcgtacctgagttttggttcttacgaaggtgcttttttcgtgtgtagatacttgtaaaatttgctgttcctgcagggaggacgattggtagaggcttctattcagccatcttgctccacttcctttgtctggcgattgctttcagaaatagctttgtgaggtcattttttgagactagtgatgaaaagcttcacagtcacagagtaacatttggcaataaattagttcagcttgtttccacatggtccccaaatcttcatttgttccatcatgaaaaacaaactttcatttgcgagtaagtctgaggctctcaaattgtctttcagaaatgtaacagaaataatggcactacctgtaacagacacacagcctaacggagcgatcagagtaatgggagcaaatccataggctgcaaagttccccgtctctcccacggccatcagcaggacaccaccccaccacagcacactcttgaagtatggccttgggtgctcttgttgtgccagctgaaggtgagaatatttctgaatatttagagaaatactgatcaccaagtttcctaaaatagccagcaaaactccaaaaaggtgaatctggttcctgcggtaccagtcgcccgagagggagccgttgccggcgcctggtgccccgtacgtgaaattcagtgacagctcgtccagggcggccgaggcggagtccccggggcccgcgggcgccaccgctgccatgaggtctcgctcccggcgctcgggctccggctcgggctgcggccgcctccccgccctgttgcaccgcgaggaggccgcgccgcagccacttcctgctc

SEQ ID NO: 13839 - RNA, 3804 nt, Homo sapiens
  source 1..3804: mol_type = other RNA
gctgggattacaggcatgagccaccatgcctggcctgtaaataaagttttactggaacacagccatgctcttctgtttacatcttgtctatggctgctttagtgctacaatggcagagttgggtagttgggacagacaccatgtctgtctgttggtacagacaacacaaactccaaaatatgtactctgtgggtctttactgaaaactttgccgacccttggtctagacagatagtcagatgagctaacagttggctaaaggtcctcaactcacaatgccaagagaaggactgagttggctttagttgttgtcatgcactgtgtaatttaaaaaatcttacaggccagtacaactaaaactcctatttaccttactttggagcaacaatatggaaagtaaaactaggtctgaatatattttatatgttacctggacttctaaaacattgttgattgcttaaatgtgcataagtcaatgtcatttctcaaaacgtttaatagatgcaactgttggcggctgctaaagtactggtgttatgcttgtgcctgtgtgaaattctacagtgctgaaaatctcatgcactctagctatgaatgcaggtctacttgaagcaaaactcttcaatctaattgttttctcaatctttgtaaaccagttttaagagtcaccagaaatctgtagtttaaggcaccagatacatttcttggctgagccttgtaggaccaatatgctggaccaattcggtaaaatacaccataaattatgactgctttatctgaatgcatgggacacttgctacgatggcgggaattattaccaggagtttaggagccagacatgggttctgtatttttcatacattggtgatcaattcaaatctctttcctttgcagccaggtttggtcagtctggccaggagtgcagattatgacaaagaacaaagctaaaagacctgagccattaaggttacagtctcaataccaccgagttaaacaacctatttaaatgcaagactattgattggaatgatattggacagacatgtcagaagtgatctgaaggctttgaaatgtcattaagggtgggacttattgttggatgttggctgcaacgaaggctacttcttttcttctcctttaaatattaggtagatcataaataacagatattattatggattctacctgcaaatgtgtcttagcagatatgtgatgaattggagtggaaaagccattcaggaaacaggaggacttgggcttcctcttgaagctcaggtttgaccactgggttgttttctatgtctacaggtttaaatggctgaaattcagttctctaatcacaactctccttttatctagaagaatttacaaagcttgaggtaatgactttgggaagaaatgatgtgtagtgaaactatcactaagaatttaaatgtgattttttagacttatatggagaataagacatataaatccacttgataaattataagatctataaaaaagacataggatattaaatttttcttcagtttcaagtatgatagaatcatacagctgaagaaaacatcaccattctagatttttattaaaaaataaacaaacattagtcctactttttgtctctaacgcttcatgaatttatgtgtcagccttgtgcaggggctgtgctaatctctgcattgttcctattttagtacatgggctactgaaacaagcagagtcctacttcttaaacttcctcttccttacacgtaaaaagcccaccagtcaaggtcttttaattttggtgtacactatcactgaatgccatttataaattctaattttaaagagacccttaattttcaaaggaggactttgatagcattagttttcagaaaagatgacttgcaattctaacttagtacttgaaaggtgagatttttatagggaggcttataaaaggtgtcttagaaaaaaaatgagcgctctcaaacctttcttttgggagtgaggttgtggggctgaagtgactttttaaagtgaagcaactgacactacccgtgggagaagccacctatgcgacctgtggccaaaccgcaaatgtatgtttctgtgcaacattcctgctagagcagccgggctctgagtaaggtgtagctggctagataatcactagggagaggtccagggtgtggggaacactccaaatcacattccatggaaatattagactgtcagagcttaggaagtccccgattgtccatagacgctgaggtgggggaaaggactgaaatgaatgctagcacatgttagcttataaaagagctgctgacacaaattgaacatgtgcaattttttaaaaaggtggtatcgaataacaggccaacagccatccttctcagcatttagacctctttcttctctccactttggctctttgttgagtcacttccatcaggcaaagttccataggataagctatgtgaatctggttgtattttgtccaacatttgtttcccaggaatatttccaaaatcaatataagactgttgcagatgttccttttctcgatttcttgtgaccaaaaatacaccaaggaatgacagaaaacacccaaaaagatatataaatacagtgagaaaaggagcaccaaggaattcctgataaaatatgatacctgcaatgatggcactgattgtaaagaaaatatgattaactggcaccactgttgtcgtattgtagagtttcgtggcttgattcaggaacttgacttggaaaacacaagatgctatcatgatgataaacatgatatagaaaatggggtaagttagttgcattttatccatcacagaaaaagtgatcatgcctgagacggcctttactgaaataacagtcaatgaggctagaattgccaccagggttagcagaatcaccatatgcttcattccttttcttttatagaaatacaggagaatgcagaaaattaatatttctaaaatcacatagatcaggaactgccatccgacaaggtaatactgtactgttcttgctgagattgcctgagttatatttggagcaaagttcaccagtaaatatgttcctgcaaatgccagtgtcgtacctggcgattgctttcagaaatagctttgtgaggtcattttttgagactagtgatgaaaagcttcacagtcacagagtaacatttggcaataaattagttcagcttgtttccacatggtccccaaatcttcatttgttccatcatgaaaaacaaactttcatttgcgagtaagtctgaggctctcaaattgtctttcagaaatgtaacagaaataatggcactacctgtaacagacacacagcctaacggagcgatcagagtaatgggagcaaatccataggctgcaaagttccccgtctctcccacggccatcagcaggacaccaccccaccacagcacactcttgaagtatggccttgggtgctcttgttgtgccagctgaaggtgagaatatttctgaatatttagagaaatactgatcaccaagtttcctaaaatagccagcaaaactccaaaaaggtgaatctggttcctgcggtaccagtcgcccgagagggagccgttgccggcgcctggtgccccgtacgtgaaattcagtgacagctcgtccagggcggccgaggcggagtccccggggcccgcgggcgccaccgctgccatgaggtctcgctcccggcgctcgggctccggctcgggctgcggccgcctccccgccctgttgcaccgcgaggaggccgcgccgcagccacttcctgctc

SEQ ID NO: 13840 - RNA, 3864 nt, Homo sapiens
  source 1..3864: mol_type = other RNA
gctgggattacaggcatgagccaccatgcctggcctgtaaataaagttttactggaacacagccatgctcttctgtttacatcttgtctatggctgctttagtgctacaatggcagagttgggtagttgggacagacaccatgtctgtctgttggtacagacaacacaaactccaaaatatgtactctgtgggtctttactgaaaactttgccgacccttggtctagacagatagtcagatgagctaacagttggctaaaggtcctcaactcacaatgccaagagaaggactgagttggctttagttgttgtcatgcactgtgtaatttaaaaaatcttacaggccagtacaactaaaactcctatttaccttactttggagcaacaatatggaaagtaaaactaggtctgaatatattttatatgttacctggacttctaaaacattgttgattgcttaaatgtgcataagtcaatgtcatttctcaaaacgtttaatagatgcaactgttggcggctgctaaagtactggtgttatgcttgtgcctgtgtgaaattctacagtgctgaaaatctcatgcactctagctatgaatgcaggtctacttgaagcaaaactcttcaatctaattgttttctcaatctttgtaaaccagttttaagagtcaccagaaatctgtagtttaaggcaccagatacatttcttggctgagccttgtaggaccaatatgctggaccaattcggtaaaatacaccataaattatgactgctttatctgaatgcatgggacacttgctacgatggcgggaattattaccaggagtttaggagccagacatgggttctgtatttttcatacattggtgatcaattcaaatctctttcctttgcagccaggtttggtcagtctggccaggagtgcagattatgacaaagaacaaagctaaaagacctgagccattaaggttacagtctcaataccaccgagttaaacaacctatttaaatgcaagactattgattggaatgatattggacagacatgtcagaagtgatctgaaggctttgaaatgtcattaagggtgggacttattgttggatgttggctgcaacgaaggctacttcttttcttctcctttaaatattaggtagatcataaataacagatattattatggattctacctgcaaatgtgtcttagcagatatgtgatgaattggagtggaaaagccattcaggaaacaggaggacttgggcttcctcttgaagctcaggtttgaccactgggttgttttctatgtctacaggtttaaatggctgaaattcagttctctaatcacaactctccttttatctagaagaatttacaaagcttgaggtaatgactttgggaagaaatgatgtgtagtgaaactatcactaagaatttaaatgtgattttttagacttatatggagaataagacatataaatccacttgataaattataagatctataaaaaagacataggatattaaatttttcttcagtttcaagtatgatagaatcatacagctgaagaaaacatcaccattctagatttttattaaaaaataaacaaacattagtcctactttttgtctctaacgcttcatgaatttatgtgtcagccttgtgcaggggctgtgctaatctctgcattgttcctattttagtacatgggctactgaaacaagcagagtcctacttcttaaacttcctcttccttacacgtaaaaagcccaccagtcaaggtcttttaattttggtgtacactatcactgaatgccatttataaattctaattttaaagagacccttaattttcaaaggaggactttgatagcattagttttcagaaaagatgacttgcaattctaacttagtacttgaaaggtgagatttttatagggaggcttataaaaggtgtcttagaaaaaaaatgagcgctctcaaacctttcttttgggagtgaggttgtggggctgaagtgactttttaaagtgaagcaactgacactacccgtgggagaagccacctatgcgacctgtggccaaaccgcaaatgtatgtttctgtgcaacattcctgctagagcagccgggctctgagtaaggtgtagctggctagataatcactagggagaggtccagggtgtggggaacactccaaatcacattccatggaaatattagactgtcagagcttaggaagtccccgattgtccatagacgctgaggtgggggaaaggactgaaatgaatgctagcacatgttagcttataaaagagctgctgacacaaattgaacatgtgcaattttttaaaaaggtggtatcgaataacaggccaacagccatccttctcagcatttagacctctttcttctctccactttggctctttgttgagtcacttccatcaggcaaagttccataggataagctatgtgaatctggttgtattttgtccaacatttgtttcccaggaatatttccaaaatcaatataagactgttgcagatgttccttttctcgatttcttgtgaccaaaaatacaccaaggaatgacagaaaacacccaaaaagatatataaatacagtgagaaaaggagcaccaaggaattcctgataaaatatgatacctgcaatgatggcactgattgtaaagaaaatatgattaactggcaccactgttgtcgtattgtagagtttcgtggcttgattcaggaacttgacttggaaaacacaagatgctatcatgatgataaacatgatatagaaaatggggtaagttagttgcattttatccatcacagaaaaagtgatcatgcctgagacggcctttactgaaataacagtcaatgaggctagaattgccaccagggttagcagaatcaccatatgcttcattccttttcttttatagaaatacaggagaatgcagaaaattaatatttctaaaatctagtttgaccttgaaaactccactcctctttgcattttggcaaggatggggattgcccatctgcagcagacaggctgggaaaggctgttttagtgagtgcactttattcttctctggctggtatacactgggcttctcaaatcttccttcctttcttttctgtaccagatcagaggaaaagctcctgagccttgtctctgtgaggcttccatttaatgtaaatcacatagatcaggaactgccatccgacaaggtaatactgtactgttcttgctgagattgcctgagttatatttggagcaaagttcaccagtaaatatgttcctgcaaatgccagtgtcgtaccgagtaagtctgaggctctcaaattgtctttcagaaatgtaacagaaataatggcactacctgtaacagacacacagcctaacggagcgatcagagtaatgggagcaaatccataggctgcaaagttccccgtctctcccacggccatcagcaggacaccaccccaccacagcacactcttgaagtatggccttgggtgctcttgttgtgccagctgaaggtgagaatatttctgaatatttagagaaatactgatcaccaagtttcctaaaatagccagcaaaactccaaaaaggtgaatctggttcctgcggtaccagtcgcccgagagggagccgttgccggcgcctggtgccccgtacgtgaaattcagtgacagctcgtccagggcggccgaggcggagtccccggggcccgcgggcgccaccgctgccatgaggtctcgctcccggcgctcgggctccggctcgggctgcggccgcctccccgccctgttgcaccgcgaggaggccgcgccgcagccacttcctgctc

SEQ ID NO: 13841 - RNA, 3545 nt, Homo sapiens
  source 1..3545: mol_type = other RNA
gctgggattacaggcatgagccaccatgcctggcctgtaaataaagttttactggaacacagccatgctcttctgtttacatcttgtctatggctgctttagtgctacaatggcagagttgggtagttgggacagacaccatgtctgtctgttggtacagacaacacaaactccaaaatatgtactctgtgggtctttactgaaaactttgccgacccttggtctagacagatagtcagatgagctaacagttggctaaaggtcctcaactcacaatgccaagagaaggactgagttggctttagttgttgtcatgcactgtgtaatttaaaaaatcttacaggccagtacaactaaaactcctatttaccttactttggagcaacaatatggaaagtaaaactaggtctgaatatattttatatgttacctggacttctaaaacattgttgattgcttaaatgtgcataagtcaatgtcatttctcaaaacgtttaatagatgcaactgttggcggctgctaaagtactggtgttatgcttgtgcctgtgtgaaattctacagtgctgaaaatctcatgcactctagctatgaatgcaggtctacttgaagcaaaactcttcaatctaattgttttctcaatctttgtaaaccagttttaagagtcaccagaaatctgtagtttaaggcaccagatacatttcttggctgagccttgtaggaccaatatgctggaccaattcggtaaaatacaccataaattatgactgctttatctgaatgcatgggacacttgctacgatggcgggaattattaccaggagtttaggagccagacatgggttctgtatttttcatacattggtgatcaattcaaatctctttcctttgcagccaggtttggtcagtctggccaggagtgcagattatgacaaagaacaaagctaaaagacctgagccattaaggttacagtctcaataccaccgagttaaacaacctatttaaatgcaagactattgattggaatgatattggacagacatgtcagaagtgatctgaaggctttgaaatgtcattaagggtgggacttattgttggatgttggctgcaacgaaggctacttcttttcttctcctttaaatattaggtagatcataaataacagatattattatggattctacctgcaaatgtgtcttagcagatatgtgatgaattggagtggaaaagccattcaggaaacaggaggacttgggcttcctcttgaagctcaggtttgaccactgggttgttttctatgtctacaggtttaaatggctgaaattcagttctctaatcacaactctccttttatctagaagaatttacaaagcttgaggtaatgactttgggaagaaatgatgtgtagtgaaactatcactaagaatttaaatgtgattttttagacttatatggagaataagacatataaatccacttgataaattataagatctataaaaaagacataggatattaaatttttcttcagtttcaagtatgatagaatcatacagctgaagaaaacatcaccattctagatttttattaaaaaataaacaaacattagtcctactttttgtctctaacgcttcatgaatttatgtgtcagccttgtgcaggggctgtgctaatctctgcattgttcctattttagtacatgggctactgaaacaagcagagtcctacttcttaaacttcctcttccttacacgtaaaaagcccaccagtcaaggtcttttaattttggtgtacactatcactgaatgccatttataaattctaattttaaagagacccttaattttcaaaggaggactttgatagcattagttttcagaaaagatgacttgcaattctaacttagtacttgaaaggtgagatttttatagggaggcttataaaaggtgtcttagaaaaaaaatgagcgctctcaaacctttcttttgggagtgaggttgtggggctgaagtgactttttaaagtgaagcaactgacactacccgtgggagaagccacctatgcgacctgtggccaaaccgcaaatgtatgtttctgtgcaacattcctgctagagcagccgggctctgagtaaggtgtagctggctagataatcactagggagaggtccagggtgtggggaacactccaaatcacattccatggaaatattagactgtcagagcttaggaagtccccgattgtccatagacgctgaggtgggggaaaggactgaaatgaatgctagcacatgttagcttataaaagagctgctgacacaaattgaacatgtgcaattttttaaaaaggtggtatcgaataacaggccaacagccatccttctcagcatttagacctctttcttctctccactttggctctttgttgagtcacttccatcaggcaaagttccataggataagctatgtgaatctggttgtattttgtccaacatttgtttccccaaaaagatatataaatacagtgagaaaaggagcaccaaggaattcctgataaaatatgatacctgcaatgatggcactgattgtaaagaaaatatgattaactggcaccactgttgtcgtattgtagagtttcgtggcttgattcaggaacttgacttggaaaacacaagatgctatcatgatgataaacatgatatagaaaatggggtaagttagttgcattttatccatcacagaaaaagtgatcatgcctgagacggcctttactgaaataacagtcaatgaggctagaattgccaccagggttagcagaatcaccatatgcttcattccttttcttttatagaaatacaggagaatgcagaaaattaatatttctaaaatcacatagatcaggaactgccatccgacaaggtaatactgtactgttcttgctgagattgcctgagttatatttggagcaaagttcaccagtaaatatgttcctgcaaatgccagtgtcgtaccgagtaagtctgaggctctcaaattgtctttcagaaatgtaacagaaataatggcactacctgtaacagacacacagcctaacggagcgatcagagtaatgggagcaaatccataggctgcaaagttccccgtctctcccacggccatcagcaggacaccaccccaccacagcacactcttgaagtatggccttgggtgctcttgttgtgccagctgaaggtgagaatatttctgaatatttagagaaatactgatcaccaagtttcctaaaatagccagcaaaactccaaaaaggtgaatctggttcctgcggtaccagtcgcccgagagggagccgttgccggcgcctggtgccccgtacgtgaaattcagtgacagctcgtccagggcggccgaggcggagtccccggggcccgcgggcgccaccgctgccatgaggtctcgctcccggcgctcgggctccggctcgggctgcggccgcctccccgccctgttgcaccgcgaggaggccgcgccgcagccacttcctgctc

SEQ ID NO: 13842 - RNA, 3668 nt, Homo sapiens
  source 1..3668: mol_type = other RNA
gctgggattacaggcatgagccaccatgcctggcctgtaaataaagttttactggaacacagccatgctcttctgtttacatcttgtctatggctgctttagtgctacaatggcagagttgggtagttgggacagacaccatgtctgtctgttggtacagacaacacaaactccaaaatatgtactctgtgggtctttactgaaaactttgccgacccttggtctagacagatagtcagatgagctaacagttggctaaaggtcctcaactcacaatgccaagagaaggactgagttggctttagttgttgtcatgcactgtgtaatttaaaaaatcttacaggccagtacaactaaaactcctatttaccttactttggagcaacaatatggaaagtaaaactaggtctgaatatattttatatgttacctggacttctaaaacattgttgattgcttaaatgtgcataagtcaatgtcatttctcaaaacgtttaatagatgcaactgttggcggctgctaaagtactggtgttatgcttgtgcctgtgtgaaattctacagtgctgaaaatctcatgcactctagctatgaatgcaggtctacttgaagcaaaactcttcaatctaattgttttctcaatctttgtaaaccagttttaagagtcaccagaaatctgtagtttaaggcaccagatacatttcttggctgagccttgtaggaccaatatgctggaccaattcggtaaaatacaccataaattatgactgctttatctgaatgcatgggacacttgctacgatggcgggaattattaccaggagtttaggagccagacatgggttctgtatttttcatacattggtgatcaattcaaatctctttcctttgcagccaggtttggtcagtctggccaggagtgcagattatgacaaagaacaaagctaaaagacctgagccattaaggttacagtctcaataccaccgagttaaacaacctatttaaatgcaagactattgattggaatgatattggacagacatgtcagaagtgatctgaaggctttgaaatgtcattaagggtgggacttattgttggatgttggctgcaacgaaggctacttcttttcttctcctttaaatattaggtagatcataaataacagatattattatggattctacctgcaaatgtgtcttagcagatatgtgatgaattggagtggaaaagccattcaggaaacaggaggacttgggcttcctcttgaagctcaggtttgaccactgggttgttttctatgtctacaggtttaaatggctgaaattcagttctctaatcacaactctccttttatctagaagaatttacaaagcttgaggtaatgactttgggaagaaatgatgtgtagtgaaactatcactaagaatttaaatgtgattttttagacttatatggagaataagacatataaatccacttgataaattataagatctataaaaaagacataggatattaaatttttcttcagtttcaagtatgatagaatcatacagctgaagaaaacatcaccattctagatttttattaaaaaataaacaaacattagtcctactttttgtctctaacgcttcatgaatttatgtgtcagccttgtgcaggggctgtgctaatctctgcattgttcctattttagtacatgggctactgaaacaagcagagtcctacttcttaaacttcctcttccttacacgtaaaaagcccaccagtcaaggtcttttaattttggtgtacactatcactgaatgccatttataaattctaattttaaagagacccttaattttcaaaggaggactttgatagcattagttttcagaaaagatgacttgcaattctaacttagtacttgaaaggtgagatttttatagggaggcttataaaaggtgtcttagaaaaaaaatgagcgctctcaaacctttcttttgggagtgaggttgtggggctgaagtgactttttaaagtgaagcaactgacactacccgtgggagaagccacctatgcgacctgtggccaaaccgcaaatgtatgtttctgtgcaacattcctgctagagcagccgggctctgagtaaggtgtagctggctagataatcactagggagaggtccagggtgtggggaacactccaaatcacattccatggaaatattagactgtcagagcttaggaagtccccgattgtccatagacgctgaggtgggggaaaggactgaaatgaatgctagcacatgttagcttataaaagagctgctgacacaaattgaacatgtgcaattttttaaaaaggtggtatcgaataacaggccaacagccatccttctcagcatttagacctctttcttctctccactttggctctttgttgagtcacttccatcaggcaaagttccataggataagctatgtgaatctggttgtattttgtccaacatttgtttccctccaagcctttctctctggggttgtgtcaggaatatttccaaaatcaatataagactgttgcagatgttccttttctcgatttcttgtgaccaaaaatacaccaaggaatgacagaaaacacccaaaaagatatataaatacagtgagaaaaggagcaccaaggaattcctgataaaatatgatacctgcaatgatggcactgattgtaaagaaaatatgattaactggcaccactgttgtcgtattgtagagtttcgtggcttgattcaggaacttgacttggaaaacacaagatgctatcatgatgataaacatgatatagaaaatggggtaagttagttgcattttatccatcacagaaaaagtgatcatgcctgagacggcctttactgaaataacagtcaatgaggctagaattgccaccagggttagcagaatcaccatatgcttcattccttttcttttatagaaatacaggagaatgcagaaaattaatatttctaaaatcacatagatcaggaactgccatccgacaaggtaatactgtactgttcttgctgagattgcctgagttatatttggagcaaagttcaccagtaaatatgttcctgcaaatgccagtgtcgtaccgagtaagtctgaggctctcaaattgtctttcagaaatgtaacagaaataatggcactacctgtaacagacacacagcctaacggagcgatcagagtaatgggagcaaatccataggctgcaaagttccccgtctctcccacggccatcagcaggacaccaccccaccacagcacactcttgaagtatggccttgggtgctcttgttgtgccagctgaaggtgagaatatttctgaatatttagagaaatactgatcaccaagtttcctaaaatagccagcaaaactccaaaaaggtgaatctggttcctgcggtaccagtcgcccgagagggagccgttgccggcgcctggtgccccgtacgtgaaattcagtgacagctcgtccagggcggccgaggcggagtccccggggcccgcgggcgccaccgctgccatgaggtctcgctcccggcgctcgggctccggctcgggctgcggccgcctccccgccctgttgcaccgcgaggaggccgcgccgcagccacttcctgctc

SEQ ID NO: 13843 - RNA, 6616 nt, Homo sapiens
  source 1..6616: mol_type = other RNA
gctgggattacaggcatgagccaccatgcctggcctgtaaataaagttttactggaacacagccatgctcttctgtttacatcttgtctatggctgctttagtgctacaatggcagagttgggtagttgggacagacaccatgtctgtctgttggtacagacaacacaaactccaaaatatgtactctgtgggtctttactgaaaactttgccgacccttggtctagacagatagtcagatgagctaacagttggctaaaggtcctcaactcacaatgccaagagaaggactgagttggctttagttgttgtcatgcactgtgtaatttaaaaaatcttacaggccagtacaactaaaactcctatttaccttactttggagcaacaatatggaaagtaaaactaggtctgaatatattttatatgttacctggacttctaaaacattgttgattgcttaaatgtgcataagtcaatgtcatttctcaaaacgtttaatagatgcaactgttggcggctgctaaagtactggtgttatgcttgtgcctgtgtgaaattctacagtgctgaaaatctcatgcactctagctatgaatgcaggtctacttgaagcaaaactcttcaatctaattgttttctcaatctttgtaaaccagttttaagagtcaccagaaatctgtagtttaaggcaccagatacatttcttggctgagccttgtaggaccaatatgctggaccaattcggtaaaatacaccataaattatgactgctttatctgaatgcatgggacacttgctacgatggcgggaattattaccaggagtttaggagccagacatgggttctgtatttttcatacattggtgatcaattcaaatctctttcctttgcagccaggtttggtcagtctggccaggagtgcagattatgacaaagaacaaagctaaaagacctgagccattaaggttacagtctcaataccaccgagttaaacaacctatttaaatgcaagactattgattggaatgatattggacagacatgtcagaagtgatctgaaggctttgaaatgtcattaagggtgggacttattgttggatgttggctgcaacgaaggctacttcttttcttctcctttaaatattaggtagatcataaataacagatattattatggattctacctgcaaatgtgtcttagcagatatgtgatgaattggagtggaaaagccattcaggaaacaggaggacttgggcttcctcttgaagctcaggtttgaccactgggttgttttctatgtctacaggtttaaatggctgaaattcagttctctaatcacaactctccttttatctagaagaatttacaaagcttgaggtaatgactttgggaagaaatgatgtgtagtgaaactatcactaagaatttaaatgtgattttttagacttatatggagaataagacatataaatccacttgataaattataagatctataaaaaagacataggatattaaatttttcttcagtttcaagtatgatagaatcatacagctgaagaaaacatcaccattctagatttttattaaaaaataaacaaacattagtcctactttttgtctctaacgcttcatgaatttatgtgtcagccttgtgcaggggctgtgctaatctctgcattgttcctattttagtacatgggctactgaaacaagcagagtcctacttcttaaacttcctcttccttacacgtaaaaagcccaccagtcaaggtcttttaattttggtgtacactatcactgaatgccatttataaattctaattttaaagagacccttaattttcaaaggaggactttgatagcattagttttcagaaaagatgacttgcaattctaacttagtacttgaaaggtgagatttttatagggaggcttataaaaggtgtcttagaaaaaaaatgagcgctctcaaacctttcttttgggagtgaggttgtggggctgaagtgactttttaaagtgaagcaactgacactacccgtgggagaagccacctatgcgacctgtggccaaaccgcaaatgtatgtttctgtgcaacattcctgctagagcagccgggctctgagtaaggtgtagctggctagataatcactagggagaggtccagggtgtggggaacactccaaatcacattccatggaaatattagactgtcagagcttaggaagtccccgattgtccatagacgctgaggtgggggaaaggactgaaatgaatgctagcacatgttagcttataaaagagctgctgacacaaattgaacatgtgcaattttttaaaaaggtggtatcgaataacaggccaacagccatccttctcagcatttagacctctttcttctctccactttggctctttgttgagtcacttccatcaggcaaagttccataggataagctatgtgaatctggttgtattttgtccaacatttgtttccctgtggagataataatcatagagaatcttttgaggtcttacagaaaaataagtcttaataatttctcctcaatctaggccacattttatcacctctcttttatactatgtgggcactctctaaagagaagagatgaatatcaaggaagaaaaggcccttgaaacgccatgtctgtagctatgtgatagcgaattgtctgtgtcagagccactatccccaccccacaggatctacatgctggccatggaaatcaggtgggtttagtctggagattcacatgaagcattcactcacctccaagcctttctctctggggttgtgtcttcttttccacgtcgaatgcatataacaacatagaaaaatagcctttgatagtgacttctaaagctactacggagcctatgcactgagctttgtgaaataaaaaatagagttaaaaataatcaggctcggtgcagtggctcacacctatcatcccagcacattgggaggccgaggcaggcgaatcatttgaggtcaggaattcgagaccagcctggccaacatggtgaaaacccacctctgctaaaaatacaaaaattagccgggcatggtggtgcctactcgggaggctgagacacgagaatcacttgaacccgggagggggaggctgcagtaagctgagattgtgccactgcactccagcctgggcaacagagcaagactccatctcaaaaaaaaaaaaaaaagtcaaactttatttcctatcaaagaacctctaaccatataaggcttctatcacaagcacctttgccactgatgccaattctttcattgactgctcccagcagataagatggctcgaatggcaaagagaacacagaattcattgcatggggccatatttctcagtcttagggatgaggcttccctagtttttgcttcacaggcatggtgctaacagaatggtggagaaagctgtgagaatgtctccactcctgcctggaaacctataggtccccctacatccccagtaaggctggagagtgctgagggcgggtggacaggggaagaggtgacacagcagacagtttcctttgtcctggacttggcttttgttgtctacatgactaggcgagttatttctcagtgagagtgagaacgggaaagagtgtttgctctctgggtaggcggggtgaggaagggggaagaaactactcatgttttggtgactgtcctgagccacagtgcacaggccacctcaggcttcccccaagacatgctccttagctgcctaccctttgtccttggatgttccttcaaggctctcaaagtggcaggggtctgctgctggtagtcattgctactcttttctctacccttttccaatttaaggaaacccaaaaaggaaatcctccaaatcacccaaatcgaggaaacatggtcagttcttttatatccccagttctgtgcaaaactgacattcaataaattattagaaacatttacactgaaaatagcacctttggtttcattattaaatgtacattttttaggataagaattatgttttatattaacttaccacccaaaataataccaataactattcatttataaggatcaaattttccactataaagaatatatgattttaccaggaatatttccaaaatcaatataagactgttgcagatgttccttttctcgatttcttgtgaccaaaaatacaccaaggaatgacagaaaacacctgtaaggataatattaataaagaatacaagaacactgaaacagactcatggtattaaataactgagctccatattctacatgatgacataaatcccattggttttgttcttccagtttctcatggtaagcttcctagtacttgtcttaattagcacagccaatagttctacccagaaccaagacttgggcagattccagtagatctctggcccaggtttttaccatctgggggctaactcaggctcaaaacccttggggacaccctgtctcattttctgcccatgcacgcccagatccatttctggcatgtgacacaagagaaaaaataatttattctttaattttctaagaaatctagttttccttggccataagagtagtcataatttccagacctcagaagtttggccttgcccaattatcttatgaaattgaattttcaagatagatggcttcctacaccgaaaatagcctaggctcaagtttgcataacaatgatcatgctgactactagatcaaggagcagctaaacatttaatgaagtgcctcatggagtcatggaagctcctatacactggtgatatattgtcaaagttctgctctctgtttgcaagcaatgctagcaatgatgcccaccaaatctctagggagagctcaagctgcacactcttaacacaagaaagggatgctaccaacctgatattatcatgactaaagcaagggatctgcccatcttggccttttattttgggcgaccctagaggatcatgattctctaatttagatctaatctaggggttcccaagagcgaagtaggtctgatacagtacagaaaggtcgtgcagtaactacaagggccagtggatgtatcttgtctttggcctggaattggaaatccccaatgtttcagaacagcagagatatacctaagtcacaaagccaaagacgctgagccctgtttagggccttaagttaaaaaatatgtttcttttaggagctcaggaaactgatgtttcttatattattttccaattttctatacctccggtacaatgccgaaaatcctacgtaaaagtaatagaatttcacatgctttacctctgagacatttactcacccaaaaagatatataaatacagtgagaaaaggagcaccaaggaattcctgataaaatatgatacctgcaatgatggcactgattgtaaagaaaatatgattaactggcaccactgttgtcgtattgtagagtttcgtggcttgattcaggaacttgacttggaaaacacaagatgctatcatgatgataaacatgatatagaaaatggggtaagttagttgcattttatccatcacagaaaaagtgatcatgcctgagacggcctttactgaaataacagtcaatgaggctagaattgccaccagggttagcagaatcaccatatgcttcattccttttcttttatagaaatacaggagaatgcagaaaattaatatttctaaaatctagtttgaccttgaaaactccactcctctttgcattttggcaaggatggggattgcccatctgcagcagacaggctgggaaaggctgttttagtgagtgcactttattcttctctggctggtatacactgggcttctcaaatcttccttcctttcttttctgtaccagatcagaggaaaagctcctgagccttgtctctgtgaggcttccatttaatgtaaatcacatagatcaggaactgccatccgacaaggtaatactgtactgttcttgctgagattgcctgagttatatttggagcaaagttcaccagtaaatatgttcctgcaaatgccagtgtcgtaccgagtaagtctgaggctctcaaattgtctttcagaaatgtaacagaaataatggcactacctgtaacagacacacagcctaacggagcgatcagagtaatgggagcaaatccataggctgcaaagttccccgtctctcccacggccatcagcaggacaccaccccaccacagcacactcttgaagtatggccttgggtgctcttgttgtgccagctgaaggtgagaatatttctgaatatttagagaaatactgatcaccaagtttcctaaaatagccagcaaaactccaaaaaggtgaatctggttcctgcggtaccagtcgcccgagagggagccgttgccggcgcctggtgccccgtacgtgaaattcagtgacagctcgtccagggcggccgaggcggagtccccggggcccgcgggcgccaccgctgccatgaggtctcgctcccggcgctcgggctccggctcgggctgcggccgcctccccgccctgttgcaccgcgaggaggccgcgccgcagccacttcct

SEQ ID NO: 13844 - RNA, 6640 nt, Homo sapiens
  source 1..6640: mol_type = other RNA
gctgggattacaggcatgagccaccatgcctggcctgtaaataaagttttactggaacacagccatgctcttctgtttacatcttgtctatggctgctttagtgctacaatggcagagttgggtagttgggacagacaccatgtctgtctgttggtacagacaacacaaactccaaaatatgtactctgtgggtctttactgaaaactttgccgacccttggtctagacagatagtcagatgagctaacagttggctaaaggtcctcaactcacaatgccaagagaaggactgagttggctttagttgttgtcatgcactgtgtaatttaaaaaatcttacaggccagtacaactaaaactcctatttaccttactttggagcaacaatatggaaagtaaaactaggtctgaatatattttatatgttacctggacttctaaaacattgttgattgcttaaatgtgcataagtcaatgtcatttctcaaaacgtttaatagatgcaactgttggcggctgctaaagtactggtgttatgcttgtgcctgtgtgaaattctacagtgctgaaaatctcatgcactctagctatgaatgcaggtctacttgaagcaaaactcttcaatctaattgttttctcaatctttgtaaaccagttttaagagtcaccagaaatctgtagtttaaggcaccagatacatttcttggctgagccttgtaggaccaatatgctggaccaattcggtaaaatacaccataaattatgactgctttatctgaatgcatgggacacttgctacgatggcgggaattattaccaggagtttaggagccagacatgggttctgtatttttcatacattggtgatcaattcaaatctctttcctttgcagccaggtttggtcagtctggccaggagtgcagattatgacaaagaacaaagctaaaagacctgagccattaaggttacagtctcaataccaccgagttaaacaacctatttaaatgcaagactattgattggaatgatattggacagacatgtcagaagtgatctgaaggctttgaaatgtcattaagggtgggacttattgttggatgttggctgcaacgaaggctacttcttttcttctcctttaaatattaggtagatcataaataacagatattattatggattctacctgcaaatgtgtcttagcagatatgtgatgaattggagtggaaaagccattcaggaaacaggaggacttgggcttcctcttgaagctcaggtttgaccactgggttgttttctatgtctacaggtttaaatggctgaaattcagttctctaatcacaactctccttttatctagaagaatttacaaagcttgaggtaatgactttgggaagaaatgatgtgtagtgaaactatcactaagaatttaaatgtgattttttagacttatatggagaataagacatataaatccacttgataaattataagatctataaaaaagacataggatattaaatttttcttcagtttcaagtatgatagaatcatacagctgaagaaaacatcaccattctagatttttattaaaaaataaacaaacattagtcctactttttgtctctaacgcttcatgaatttatgtgtcagccttgtgcaggggctgtgctaatctctgcattgttcctattttagtacatgggctactgaaacaagcagagtcctacttcttaaacttcctcttccttacacgtaaaaagcccaccagtcaaggtcttttaattttggtgtacactatcactgaatgccatttataaattctaattttaaagagacccttaattttcaaaggaggactttgatagcattagttttcagaaaagatgacttgcaattctaacttagtacttgaaaggtgagatttttatagggaggcttataaaaggtgtcttagaaaaaaaatgagcgctctcaaacctttcttttgggagtgaggttgtggggctgaagtgactttttaaagtgaagcaactgacactacccgtgggagaagccacctatgcgacctgtggccaaaccgcaaatgtatgtttctgtgcaacattcctgctagagcagccgggctctgagtaaggtgtagctggctagataatcactagggagaggtccagggtgtggggaacactccaaatcacattccatggaaatattagactgtcagagcttaggaagtccccgattgtccatagacgctgaggtgggggaaaggactgaaatgaatgctagcacatgttagcttataaaagagctgctgacacaaattgaacatgtgcaattttttaaaaaggtggtatcgaataacaggccaacagccatccttctcagcatttagacctctttcttctctccactttggctctttgttgagtcacttccatcaggcaaagttccataggataagctatgtgaatctggttgtattttgtccaacatttgtttccctgtggagataataatcatagagaatcttttgaggtcttacagaaaaataagtcttaataatttctcctcaatctaggccacattttatcacctctcttttatactatgtgggcactctctaaagagaagagatgaatatcaaggaagaaaaggcccttgaaacgccatgtctgtagctatgtgatagcgaattgtctgtgtcagagccactatccccaccccacaggatctacatgctggccatggaaatcaggtgggtttagtctggagattcacatgaagcattcactcacctccaagcctttctctctggggttgtgtcttcttttccacgtcgaatgcatataacaacatagaaaaatagcctttgatagtgacttctaaagctactacggagcctatgcactgagctttgtgaaataaaaaatagagttaaaaataatcaggctcggtgcagtggctcacacctatcatcccagcacattgggaggccgaggcaggcgaatcatttgaggtcaggaattcgagaccagcctggccaacatggtgaaaacccacctctgctaaaaatacaaaaattagccgggcatggtggtgcctactcgggaggctgagacacgagaatcacttgaacccgggagggggaggctgcagtaagctgagattgtgccactgcactccagcctgggcaacagagcaagactccatctcaaaaaaaaaaaaaaaagtcaaactttatttcctatcaaagaacctctaaccatataaggcttctatcacaagcacctttgccactgatgccaattctttcattgactgctcccagcagataagatggctcgaatggcaaagagaacacagaattcattgcatggggccatatttctcagtcttagggatgaggcttccctagtttttgcttcacaggcatggtgctaacagaatggtggagaaagctgtgagaatgtctccactcctgcctggaaacctataggtccccctacatccccagtaaggctggagagtgctgagggcgggtggacaggggaagaggtgacacagcagacagtttcctttgtcctggacttggcttttgttgtctacatgactaggcgagttatttctcagtgagagtgagaacgggaaagagtgtttgctctctgggtaggcggggtgaggaagggggaagaaactactcatgttttggtgactgtcctgagccacagtgcacaggccacctcaggcttcccccaagacatgctccttagctgcctaccctttgtccttggatgttccttcaaggctctcaaagtggcaggggtctgctgctggtagtcattgctactcttttctctacccttttccaatttaaggaaacccaaaaaggaaatcctccaaatcacccaaatcgaggaaacatggtcagttcttttatatccccagttctgtgcaaaactgacattcaataaattattagaaacatttacactgaaaatagcacctttggtttcattattaaatgtacattttttaggataagaattatgttttatattaacttaccacccaaaataataccaataactattcatttataaggatcaaattttccactataaagaatatatgattttaccaggaatatttccaaaatcaatataagactgttgcagatgttccttttctcgatttcttgtgaccaaaaatacaccaaggaatgacagaaaacacctgtaaggataatattaataaagaatacaagaacactgaaacagactcatggtattaaataactgagctccatattctacatgatgacataaatcccattggttttgttcttccagtttctcatggtaagcttcctagtacttgtcttaattagcacagccaatagttctacccagaaccaagacttgggcagattccagtagatctctggcccaggtttttaccatctgggggctaactcaggctcaaaacccttggggacaccctgtctcattttctgcccatgcacgcccagatccatttctggcatgtgacacaagagaaaaaataatttattctttaattttctaagaaatctagttttccttggccataagagtagtcataatttccagacctcagaagtttggccttgcccaattatcttatgaaattgaattttcaagatagatggcttcctacaccgaaaatagcctaggctcaagtttgcataacaatgatcatgctgactactagatcaaggagcagctaaacatttaatgaagtgcctcatggagtcatggaagctcctatacactggtgatatattgtcaaagttctgctctctgtttgcaagcaatgctagcaatgatgcccaccaaatctctagggagagctcaagctgcacactcttaacacaagaaagggatgctaccaacctgatattatcatgactaaagcaagggatctgcccatcttggccttttattttgggcgaccctagaggatcatgattctctaatttagatctaatctaggggttcccaagagcgaagtaggtctgatacagtacagaaaggtcgtgcagtaactacaagggccagtggatgtatcttgtctttggcctggaattggaaatccccaatgtttcagaacagcagagatatacctaagtcacaaagccaaagacgctgagccctgtttagggccttaagttaaaaaatatgtttcttttaggagctcaggaaactgatgtttcttatattattttccaattttctatacctccggtacaatgccgaaaatcctacgtaaaagtaatagaatttcacatgctttacctctgagacatttactcacccaaaaagatatataaatacagtgagaaaaggagcaccaaggaattcctgataaaatatgatacctgcaatgatggcactgattgtaaagaaaatatgattaactggcaccactgttgtcgtattgtagagtttcgtggcttgattcaggaacttgacttggaaaacacaagatgctatcatgatgataaacatgatatagaaaatggggtaagttagttgcattttatccatcacagaaaaagtgatcatgcctgagacggcctttactgaaataacagtcaatgaggctagaattgccaccagggttagcagaatcaccatatgcttcattccttttcttttatagaaatacaggagaatgcagaaaattaatatttctaaaatctagtttgaccttgaaaactccactcctctttgcattttggcaaggatggggattgcccatctgcagcagacaggctgggaaaggctgttttagtgagtgcactttattcttctctggctggtatacactgggcttctcaaatcttccttcctttcttttctgtaccagatcagaggaaaagctcctgagccttgtctctgtgaggcttccatttaatgtaaatcttgaaggaaaaacagacatctgtcacatagatcaggaactgccatccgacaaggtaatactgtactgttcttgctgagattgcctgagttatatttggagcaaagttcaccagtaaatatgttcctgcaaatgccagtgtcgtaccgagtaagtctgaggctctcaaattgtctttcagaaatgtaacagaaataatggcactacctgtaacagacacacagcctaacggagcgatcagagtaatgggagcaaatccataggctgcaaagttccccgtctctcccacggccatcagcaggacaccaccccaccacagcacactcttgaagtatggccttgggtgctcttgttgtgccagctgaaggtgagaatatttctgaatatttagagaaatactgatcaccaagtttcctaaaatagccagcaaaactccaaaaaggtgaatctggttcctgcggtaccagtcgcccgagagggagccgttgccggcgcctggtgccccgtacgtgaaattcagtgacagctcgtccagggcggccgaggcggagtccccggggcccgcgggcgccaccgctgccatgaggtctcgctcccggcgctcgggctccggctcgggctgcggccgcctccccgccctgttgcaccgcgaggaggccgcgccgcagccacttcct

SEQ ID NO: 13845 - RNA, 2012 nt, Homo sapiens
  source 1..2012: mol_type = other RNA
gctgggattacaggcatgagccaccatgcctggcctgtccagttttgtatttaagtagcataaatacaaacataatatgtaaacataatacctacttattgtgagctattacacattctgcattctatgaagcaatttacatcatcgatcacatttaactctcacaactttatgaagtggtatcatccccattttacaggaaatggaggctcagggagagcaagtgtcccaaccatgatccctgagtggagctgtggcagagcaggaattttatgtcggatgtgtctgttccaaagcccaatctcccactgcaccccctactcccttacactctcctctattcctcggaatctctctgaacacagttcccaaagctgctcctctccgtgggatttaaggaacattagacatgctcactgcactttgctgcttggttttttggatcccgaatgtcttgggaagccttttctggtgccacttgtcttttgcttgttcttcttgaagaccttattcacccagtttgagtcttcagcagggctctccgttacataaggcttgctgacggtttccttcacatgaaccagaggcacggcgctttttggttttgaagagacaagaagagctacagcttggggctgttcttggcctagttcctccacaggtggctgagcagggaaggctgaaagagaacttcggggcagtgtttgaggtgcccccacagttgaaggccccagggatggcctgggtgaagtgggtgcctgagagtgtagggatctggctggtgatccagacggttgtacctgctgctgaggtgacagaggtgacagtccaggtggtggggtgggcagtgatgaaccaggtgtggagctgggtggcttgtgcacagctgggaatgatacaggtggcatgccacttagagaaagtggagttgaagaggccagtggctgtgcaggtggctgctcaagtggagagactggtgctgaaacaggtgactcgcatgtgaattcaagtgtctgcacaggttgggacacaggcggaccatggctgccccttccatcccctttgggaacccactccttgtgaggttgtgtggctccttccagactggcctgccgtgctcgaaggcttggttgactgcgttcagggcactcattgccaagggcgagttctatctggcagtacacttccacccgggggaaaatcactctcttggaggaagaattaagataaacagcattcagccgcctcaagtacaaaactgcatcctcgtaccctcggtagtagtaatcgtgcaggatcaccaggtccggggggaacaatgcgtgggtcatcctggcgatgttctccagggagaactggaaggagcagttgaacatgcggaagtcgtggaagatggccgggcagtcccggggacagatgtcctgctgcccactgaaggtggagatggtgatggcgtcggtccagaaggcacagggctgcatgcccgtgaagcccccatcgatgtacctcacaccgcggtaagtcggggggatgaggccacagtacaccgggacgaagcagctgcagtatagggcctcaatgagctcctccttggacgtgaactctgaaaccaccacattctccccgtccgttaagcgggtgaggctcacatggagcttccccgtggtgaccttgtaggagtcctcgggcaggacccggtacagaaactgcctcatcatctgcaccatcttacaggacggggacaagggccccaggaaggatttcttcacctcggccacacccacgttgaggactctgagatactcatccatttcaatcccgcagatggccagggcggcgatcacagcacctgccgatgtccccgcaaagcggtgggctgtttccagcatccggggggccaggtcccgcagggcgtccacagcccccgcctggtagaaggagaggaatccactgcccgagaaggagatggagtgaggggtgtccgggtcccccttgaacacctgttcttccat

SEQ ID NO: 13846 - RNA, 1901 nt, Homo sapiens
  source 1..1901: mol_type = other RNA
gctgggattacaggcatgagccaccatgcctggcctgtccagttttgtatttaagtagcataaatacaaacataatatgtaaacataatacctacttattgtgagctattacacattctgcattctatgaagcaatttacatcatcgatcacatttaactctcacaactttatgaagtggtatcatccccattttacaggaaatggaggctcagggagagcaagtgtcccaaccatgatccctgagtggagctgtggcagagcaggaattttatgtcggatgtgtctgttccaaagcccaatctcccactgcaccccctactcccttacactctcctctattcctcggaatctctctgaacacagttcccaaagctgctcctctccgtgggatttaaggaacattagacatgctcactgcactttgctgcttggttttttggatcccgaatgtcttgggaagccttttctggtgccacttgtcttttgcttgttcttcttgaagaccttattcacccagtttgagtcttcagcagggctctccgttacataaggcttgctgacggtttccttcacatgaaccagaggcacggcgctttttggttttgaagagacaagaagagctacagcttggggctgttcttggcctagttcctccacaggtggctgagcagggaaggctgaaagagaacttcggggcagtgtttgaggtgcccccacagttgaaggccccagggatggcctgggtgaagtgggtgcctgagagtgtagggatctggctggtgatccagacggttgtacctgctgctgaggtgacagaggtgacagtccaggtggtggggtgggcagtgatgaaccaggtgtggagctgggtggcttgtgcacagctgggaatgatacaggtggcatgccacttagagaaagtggagttgaagaggccagtggctgtgcaggtggctgctcaagtggagagactggtgctgaaacaggtgactcgcatgtgaattcaagtgtctgcacaggttgggacacaggcggaccatggctgccccttccatcccctttgggaacccactccttgtgaggttgtgtggctccttccagactggcctgccgtgctcgaaggcttggttgactgcgttcagggcactcattgccaagggcgagttctatctggcagtacacttccacccgggggaaaatcactctcttggaggaagaattaagataaacagcattcagccgcctcaagtacaaaactgcatcctcgtaccctcggtagtagtaatcgtgcaggatcaccaggtccggggggaacaatgcgtgggtcatcctggcgatgttctccagggagaactggaaggagcagttgaacatgcggaagtcgtggaagatggccgggcagtcccggggacagatgtcctgctgcccactgaaggtggagatggtgatggcgtcggtccagaaggcacagggctgcatgcccgtgaagcccccatcgatgtacctcacaccgcggtaagtcggggggatgaggccacagtacaccgggacgaagcagctgcagtatagggcctcaatgagctcctccttggacgtgaactctgaaaccaccacattctccccgtccgttaagcgggtgaggctcacatggagcttccccgtggtgaccttgtaggagtcctcgggcaggacccggtacagaaactgcctcatcatctgcaccatcttacaggacggggacaagggccccaggaaggatttcttcacctcggccacacccacgttgaggactctgagatactcatcttagtagaagcagctcaatcatctcctcctccaagaagccttccattgtggactgccctccaatgtgggctccccctggctgattttgtgtct

SEQ ID NO: 13847 - RNA, 2674 nt, Homo sapiens
  source 1..2674: mol_type = other RNA
gctgggattacaggcatgagccaccatgcctggcctgtccagttttgtatttaagtagcataaatacaaacataatatgtaaacataatacctacttattgtgagctattacacattctgcattctatgaagcaatttacatcatcgatcacatttaactctcacaactttatgaagtggtatcatccccattttacaggaaatggaggctcagggagagcaagtgtcccaaccatgatccctgagtggagctgtggcagagcaggaattttatgtcggatgtgtctgttccaaagcccaatctcccactgcaccccctactcccttacactctcctctattcctcggaatctctctgaacacagttcccaaagctgctcctctccgtgggatttaaggaacattagacatgctcactgcactttgctgcttggttttttggatcccgaatgtcttgggaagccttttctggtgccacttgtcttttgcttgttcttcttgaagaccttattcacccagtttgagtcttcagcagggctctccgttacataaggcttgctgacggtttccttcacatgaaccagaggcacggcgctttttggttttgaagagacaagaagagctacagcttggggctgttcttggcctagttcctccacaggtggctgagcagggaaggctgaaagagaacttcggggcagtgtttgaggtgcccccacagttgaaggccccagggatggcctgggtgaagtgggtgcctgagagtgtagggatctggctggtgatccagacggttgtacctgctgctgaggtgacagaggtgacagtccaggtggtggggtgggcagtgatgaaccaggtgtggagctgggtggcttgtgcacagctgggaatgatacaggtggcatgccacttagagaaagtggagttgaagaggccagtggctgtgcaggtggctgctcaagtggagagactggtgctgaaacaggtgactcgcatgtgaattcaagtgtctgcacaggttgggacacaggcggaccatggctgccccttccatcccctttgggaacccactccttgtgaggttgtgtggctccttccagactggcctgccgtgctcgaaggcttggttgactgcgttcagggcactcattgccaagggcgagttctatctggcagtacacttccacccgggggaaaatcactctcttggaggaagaattaagataaacagcattcagccgcctcaagtacaaaactgcatcctcgtaccctcggtagtagtaatcgtgcaggatcaccaggtccggggggaacaatgcgtgggtcatcctggcgatgttctccagggagaactggaaggagcagttgaacatgcggaagtcgtggaagatggccgggcagtcccggggacagatgtcctgctgcccactgaaggtggagatggtgatggcgtcggtccagaaggcacagggctgcatgcccgtgaagcccccatcgatgtacctctgtgggggcagagtgagaaatgcccacacaccgcggtaagtcggggggatgaggccacagtacaccgggacgaagcagctgcagtatagggcctcaatgagctcctccttggacgtgaactctgaaaccaccacattctccccgtccgttaagcgggtgaggctcacatggagcttccccgtggtgaccttgtaggagtcctcgggcaggacccggtacagaaactgcctcatcatctgcaccatcttacaggacggggacaagggccccaggaaggatttcttcacctcggccacacccacgttgaggactctgagatactcatccatttcaatcccgcagatggccagggcggcgatcacagcacctgccgatgtccccgcaaagcggtgggctgtttccagcatccggggggccaggtcccgcagggcgtccacagcccccgcctggtagaaggagaggaatccactgcccgagaaggagatggagtgaggggtgtccgggtcccccttgaacacctgttcttccatctcctcggcctctgactttctgcggaaggcggagccacccttcagcacttgcctgcccgagcctgggctgccgctccctgtaggaactccctacccagcttccctgccaccccggagcttggaatgtggctgtctctacccggctggagcaaccacaggctgctcaggaagctgcctcagcctgttaagctccgccaggaggcaactccaaaggttggaaaggggccccagaatgagatgcagaaggctcccccggtgtgtgagcagggtcttggtcctgtgagccccccactggcttcatttcttggctagattcatctcgggcacgggatcctcagccctctgcccatccatggtataccagggcgcattcactgctccccagcacagggccatgcccaaggaggcgggctctgcccagccctcagctgcaacattcagttgcaaaacctccgtgatggttatcggtgtacacctccctccccaacatgctgctgcggccgtgaagggcttccaagcccgcctccctccaggaggacggtgcctaccccatctcttttggacgggtcccccaaaagagatgcccctcctgggctccttcaggctatgtggtatgtgtgatgtgttacacaagc

SEQ ID NO: 13848 - RNA, 1928 nt, Homo sapiens
  source 1..1928: mol_type = other RNA
gctgggattacaggcatgagccaccatgcctggcctgtccagttttgtatttaagtagcataaatacaaacataatatgtaaacataatacctacttattgtgagctattacacattctgcattctatgaagcaatttacatcatcgatcacatttaactctcacaactttatgaagtggtatcatccccattttacaggaaatggaggctcagggagagcaagtgtcccaaccatgatccctgagtggagctgtggcagagcaggaattttatgtcggatgtgtctgttccaaagcccaatctcccactgcaccccctactcccttacactctcctctattcctcggaatctctctgaacacagttcccaaagctgctcctctccgtgggatttaaggaacattagacatgctcactgcactttgctgcttggttttttggatcccgaatgtcttgggaagccttttctggtgccacttgtcttttgcttgttcttcttgaagaccttattcacccagtttgagtcttcagcagggctctccgttacataaggcttgctgacggtttccttcacatgaaccagaggcacggcgctttttggttttgaagagacaagaagagctacagcttggggctgttcttggcctagttcctccacaggtggctgagcagggaaggctgaaagagaacttcggggcagtgtttgaggtgcccccacagttgaaggccccagggatggcctgggtgaagtgggtgcctgagagtgtagggatctggctggtgatccagacggttgtacctgctgctgaggtgacagaggtgacagtccaggtggtggggtgggcagtgatgaaccaggtgtggagctgggtggcttgtgcacagctgggaatgatacaggtggcatgccacttagagaaagtggagttgaagaggccagtggctgtgcaggtggctgctcaagtggagagactggtgctgaaacaggtgactcgcatgtgaattcaagtgtctgcacaggttgggacacaggcggaccatggctgccccttccatcccctttgggaacccactccttgtgaggttgtgtggctccttccagactggcctgccgtgctcgaaggcttggttgactgcgttcagggcactcattgccaagggcgagttctatctggcagtacacttccacccgggggaaaatcactctcttggaggaagaattaagataaacagcattcagccgcctcaagtacaaaactgcatcctcgtaccctcggtagtagtaatcgtgcaggatcaccaggtccggggggaacaatgcgtgggtcatcctggcgatgttctccagggagaactggaaggagcagttgaacatgcggaagtcgtggaagatggccgggcagtcccggggacagatgtcctgctgcccactgaaggtggagatggtgatggcgtcggtccagaaggcacagggctgcatgcccgtgaagcccccatcgatgtacctctgtgggggcagagtgagaaatgcccacacaccgcggtaagtcggggggatgaggccacagtacaccgggacgaagcagctgcagtatagggcctcaatgagctcctccttggacgtgaactctgaaaccaccacattctccccgtccgttaagcgggtgaggctcacatggagcttccccgtggtgaccttgtaggagtcctcgggcaggacccggtacagaaactgcctcatcatctgcaccatcttacaggacggggacaagggccccaggaaggatttcttcacctcggccacacccacgttgaggactctgagatactcatcttagtagaagcagctcaatcatctcctcctccaagaagccttccattgtggactgccctccaatgtgggctccccctggctgattttgtgtct

SEQ ID NO: 13849 - RNA, 1847 nt, Homo sapiens
  source 1..1847: mol_type = other RNA
gctgggattacaggcatgagccaccatgcctggccttcttcatagtgcctttagtaccagtactgtgtatactaagacagattctttagtactactacatagtactggtactaaagacagattctttagtactactacatagtactggtactaaagacagattctttagcactactacatagtactggtactaaagacagattctttagtactactacatagtactggtactaaagacagattctttagtactactacatagtactggtactaaagacagattctttagtactacttcatacatagtactggtactaaagattaacaacagcagcagcaacacaactggacactcctgtaggtctttgcggttgacgaagcaccttcgcatacatcatctcacggtgtccccttgaggttagtagaaaagtttgtgttatcctcactttgctgaagagaaaactgaagctcaaagcaatggagtgactttctaggttacccagaaagaaacagtaccaagatccagaaagtgcttatttttggcttggacagtttgggtaatttccaaattcacacagctggaaagtggaggtggtgagattctagaactcgtgttcttaaccacttccccaatatttagtcctgaagcattaaaaatggttttcttgttgttgctgttgttgttttagagcctgggtctcactgtgttgcccaggctggaatgcggtgcctattcacaggcgcaacaatcatggctcactgcagcctcgaactcctgggctcaagccatcctcccatctcgacctcccgagtagctgggattacaggtgcatgccaccgtgcctggcttgaaaatggtttttacacaactttgcatgatttgttcatcctgggatgaatttatatccccaaagcactggagccctggacttgtcatttgtaaccagatgatgccctcttcagctttactcttctccagttctctgagactgtgaggtccgggcactgtccattccaactccgacatgtcagccatggctgaatcagtgcttctccatccatcttcttttcacatcggaattgctagaggagtttagacagacgtacggcaggacagagagtgtttctgagaagcatcctcctttgggtctaagattgatcccatgttctgagactctattgtaaggaaacagaggtggtgccaatattaggaggcaaggagtgtcagggcagaggccagtatttaaagaagtatttcctcaaaatattggagtagtttttttttgttttgttttgtttttcctcaaaacacactgcagtcattaaccccacaaaggaagtctgctgacttcagtgagcagcatcatgatcgttcttactgaaaatggtgaagcaagccaggcaagcacctgtagtcccagctacttgggaggcggaggcaggaggatcgcttgagccaggaaattggagtccatcctgggcaacacagaaagacctcctgtctttaaaacaaacaaacaaaaaacgatgaaacagcttcacttgggatactgggtatgtctaaggaggtcagctaggagtcagtcggtttgtcaaaggccatttagacaaagattaatttacagcataaccaattcacagagtggacttgtttggtgtcattttgtctccataacagcattttaaggactagtttgtctttgtctctgctccttgctgttctagttggagtccgaaggaaaggaaaaaggaaagactgggtagacataagaacataatcttcaatttgaagaattcttatcagtgtatactttttttttctttttttttttttttttttgagacag

SEQ ID NO: 13850 - RNA, 3408 nt, Homo sapiens
  source 1..3408: mol_type = other RNA
gctgggattacaggcatgagccaccatgcctggcctttcatccatctttaaacaaattcaatgaccatctagagacagatgtgaccaaagtgttacaaatttctatgcattttctatgaattgctctgtgcagttcacacatgggttcattcaccccgcaggctgtgaacttccttatcctgtaggctgcaggtacttaggtttcagcaactacgcgacccaaaagactaaaggaggacttgtttaaattagtccctctcaaaaattgtttccaatcttataacaaacagatttaatatgcttgtgggttaaattttaaagtagttatgaagccatttactctaatataaatgaatgaaatgtaattaagaaccatacttaaacgagtacttaattttaatgaatggtatttttcatttatatacaaaggaatagccagcagcatttaaatatagaaatagtcccatctcttctctattcccttttataaagtgccattttaattgggtagatttactacccagattttcagtaactacaggataggtatctaattgtcaagaaaagcttggaaaattaagtttagcattttaaacatttgtaaaacattgctacaagtcatagagactaccaatgtattaaaataaaaagtgtaccttacataagaatcattaagttggtttaataattacttcacagaaacatgggctcatgaatacttaggccaatttgtgctaattatttaaaccagaaacagtttctgtaggtaattcagctctaagcaccattaaatagggttatgccaaatagaacaatggttaaataatcctcagaataaacaccccagcaaattcaaacttttagaatagtaacaaaagttagtgagaatccgaaagagaggcaacattttattgaaaactatcataggctgctaagtgttctctttaaataaaattttgtgtagttattaatgtaccttaacactggtgtaccttaatagtggtgttagagataggtggaaaccatactacagaagtgaatgttgcctgtttcttttgttcagtgattaaaactgaaattgcttttaaaaaaataatttaactgctacttacaatacacataaaataccaagaagattcccattttattcacattattctctaattagtatttttgcatttcaactttgatctgaccttcagtagtaccttaaaatgcaaatgcaattagtaaaaacggggcagcctgtcgttttcacacttagaaatacaatgtagtttcattacagtttgcatttttttgttactcttgaaagagtaaccccttataaaatcagatacataaaaactgcattattccttactttgcaggcatccaggaatggttaaagcaaaggaactctcattcattaattcattcattctgttcccccaatttagatacatttctagtctccagaaacggactccagggcagggaagtggagggcagagaagaggtacaggtcaaggtatgatgaatctctgaaaaagacatccacttttcccagaaggctagcctgaagagaactccgccccatccattccgatccctcaagtaagaatgcataatttagcttgtccttctggtctcacttccttacaacacctagtattcaatttattaagacaaataaacctttgcattttctaaaagaagcaatttttacccaaatacattggactttggtctcaatgtgaagggcgagtggcctttaacaggtcgttcctcccccactccctcctcccccctgccctccagcggctgctctgggtccctgaaagagggtgtggtgtggacgatctgggttctgaatcggattttgttgagtctgggttttatacgtccactagagctgcccgaggctttgcgccctggatccttggctttgcctccgacccacccctcagccgagtggtgatggtggtgatggtcccctccatcttctagggcgtgtgagagtttgtaggtgatgagatgcgagggaagcacctttgaaagcctccagcgcccgccgccgctacccgcggcgctttccccgtcaccctcgtccagggctcccaccaggttcttgatctcctcggcgatgctccgactcaggtactgggaggcctttttcccactgtagtccctgatgtccacatcggcgtcgtaggcccccaccagcagcttcaccacctccacgtggccgtgcatggctgccaagtgcagggcggtgtaacccccgctcgtcctggcgtcgatgttcaccggcagctggtgtttgttggcgaagttgactagcatggccagaagctcctgcctgccgtgcttggcggcccagtgcaggcaagtgaagccggtaatgaagtcccgcttgaccagcaggccgggctcgcaggtgagcaagccctccaggctgtcccacttgccatcggaggcagagagcatccacgcgtgctccagggggtccagcgtcacggagcctccgccgctgctctcctcctccgcggacgacgaggccaccgatgcgctgtctgagtcgcccccgcctctgccgcgtcctcccccggaggagctgcccgggctgctgcccccgggacacacgctcctcttcagctgcggggagctgcccatcaccaggtcacggaggttctggcgggccggcctctgtgcggtagcccccacaagggagctgcccctgtccgcctcctcgcagccatgtggcgggagctccaggtcctcgctgggccccggggctggagtccgcggtaggggctgcacgtcgcgccgcgagttcttcctgcgagccccggcgctcaggggcggccagtgcgcgggggcggggggctctccctcgcccagctcgcggccctgtccagggagcgactccggggccgccgcgtcggggagccgatcgcgcgcctcgggcccggcagggccgtcgggggcctcgggctcggcggtcacctggattcgcggcgggtccccggagggctcggacggcccttcacagaacctcttcttgaggtgcacgtacttggcgccgtcggcgggatcgacgcgcacagtggccacggcgttcaccagctccttgaagtgcgcgcgggcgcgggcgcgctgctccggttcgccgcctagggcgcccctgaagtgctgcaccagctcggcgtgcagggcccggcccccgcgctccgccaggaagcgcagcaccgcctcggggcccagcgccgcctcggggccccactctgccggcccctccatcctcgaccgcgctgctcccccgccagcgggcggctcagcgcggtcccatagcgacgggctcccagcggccggctcccgacggcggcggagtctggcgggctcagcgggctgccagcctacgcgtct

SEQ ID NO: 13851 - RNA, 3634 nt, Homo sapiens
  source 1..3634: mol_type = other RNA
gctgggattacaggcatgagccaccatgcctggctaaacatgtacttttttttttttttgagacaaagaaagagtcctgctctgtcgcccaggctggagtgcagtggcacaatctcagctcactgcaacctctgcctcccgggttcaagcgattcttgtgccttagcctcccaagtagctgggattacaggcacctgccaccatgcccggctaataattttttttgtatttttagtagcgatgaggtttccccatgttggccaggctggtctcaaactcctggcctcaagtgatccacccacctaggcctcccaaagtgctgggattacaggcgtgagccactgcacccggcctagttattgtttttaaaatgttagctttgtgataccatcccaaaaagtcatttattgttttttgtttgtttgggtaggagaattcatcaaagtggacattctataaatttttggttaacaaattggctcaagtcacattcttggcccaaagaccatttttggttttactttcacaggaaatacatatgaaaaagttaggtttgtggctgtcaaactgtcagctgtttttaaaatgtaatttttagtaccaccttaatactaccttataaagaatgcagaatatacttttgtatttggctttcttaaagtgaagagataatgctttaaagctaacctgctcacaaatagctgagaaatttaaaaggagattttacttaacattaactttttttaagctaaaagctcataattttaacatttggcttttctactaccctactgctgaacagagcaataaaaaaaactatactattttatttggacaatactaatataaatccttaacctataatggaaacttccaaacatgaactctaaaacatgggcatttttaatgactaccacttttaataaatatactaaaatattcaatatttgcacatcattaaataaaaaattaatttttaacaaaattttatttagagcattaggaaaatcatattcaaaacacagaaataatcagactataacaatgctgcatagatagtggtatacaagttccctgactctaacttcttcctaacttaaaagttcaattttcaagtcaccaggtagaaaatggtggaggcattatttcctctttctgaggctataaaaaaatggcttcaatggtgagaaggcaaaccatttaaacaatgaagattagattataccccaatttaattctattcccttcttgtttgttatttctcatagatgaaaatttagaatgtaataattattggaaaggaataagaagtgaattacctcttaggagataccctgatcagtgcctgctttaatcagacaaaacactaagttttaaaaattacaaccacaatattatgcctaactaaaattgccaatatgaatacttttttacagaatacattacatgtataccagaagagaaatacttgtttcctatcctctgaccttcagtagaaaaaaaatgttatcactaacaaggatcagaaaaataattttcaaggcagagcattaactcaatggggatcaaaatcttttctgaatacttaaaatagactgagtcagtcaacgagaaattgctaaatttcttctatgagagtacttttcaaaaaggaagacaatttattggaagaatttgtagctggaaacactgttcattaagaaaacattaagttaccctgagaaagactcttaatattaccagtgttttcagggccccctgaccaacgcatggaagagcaacttgtaggctctagccttttaacaatacctacataaagaatattttgatctaaaatgtaacttgggttctctgccacactggtaataagtcacaaccaagacatctgaatgtgatggagtataagcaaattttgcgtttattttaggctgccctctttcttttctaagagaaagagtttgcagttcttcaaatggtcttggatgaaacctactgtttggaaaaaagaatcttctgtaagtaaactggtagttttcttaaaacagtaaacaaatttatctggtctacattctctaaactattattatatgcctagaaaataaggcattagtaattcatcattgaccattgcagagcatagacaactgtttctttctaatcaggaccataagcaaacattcctgaaagtgcagtgttatttttaacgtctcttatgcatttacagtaagcatttgactccctacatactttcattataaaatgttttttcccaacgccttatatataccataattacttaagaaaagacaaagtgagagcagctacagaagtagcaaggtattttccacaaataaaaatacagcatacaaaaaatggcaagttagtgataattggtagtatgagtgcttattaatatcccgctttggggtccaaattaagatttgacaagtttgaagccttgtcctgtgtccagcacagtaggaagaaaccaactcatttttaatcttttcaagcacctaaaacaagttttgcagatccaaaaaaggttcagaccgcataaccaatttgccaaatgcactaggggatatgtaatacgaggaaagtgtaacatccagtgcttggccacatcgcttcccgttggcaaatgcagagtgtagtcactccaccgttttgacacaccatatactgctttcactgtgcgtcccttttcagtccagcagatgttattactggagttgcagttatattctacccagtcttttgtaaagtcacctagctgtggcgggtcagcttcttcaatatctactgtttttatcaactctgctccttgcactgcaatatactggtcattaattttcctcacttctttcacccaaggggttgaattttcgctgtctaatacgataataagccgggaacaaaaggaaccattcttttctctccaccattctataagtgtgtcaaggcgtagtgtatctccacctgctagagcccactctcctgtaccatgggtgtgcccactgtaatacaaaatatacgtatcatgtctgggtccatccactgtccgaagttcgaggaaagcttttagtttggaatgcagagtatcaaatgacagtccacttgtggaatagtcacatccataggtctcaatcatatgatatgcaaaaaatctttggatagcattgagcatgccagtagacctcaaatttaactcctgtacatgttctgggggaagcagtgttggctgaccatcaggactgcagaagttggtgggaatcacaatagcatatccaacagatgttcctcctaaacagttacccaattcatggaagagcccatgagccatggattccaatggcaaaacgattagaaacatgctcaagaaaattccatttgttggctgactcggccgtcgccaccaacgcgctctcccaaccctcggagtcagttccaaaaccaaaccaaaaaggaggagagcagacaaggcttcagcctgcgactgagaacagggaggcggcacgccttggggaacgagggcccgaggccatacgcgctaatacaggccagtgtcggcgtaaactttctccgttaccggcccggccgcgaccgccatgtttccgccgccgaaatccgc

SEQ ID NO: 13852 - RNA, 4890 nt, Homo sapiens
  source 1..4890: mol_type = other RNA
gctgggattacaggcatgagccaccatgcctggctaaacatgtacttttttttttttttgagacaaagaaagagtcctgctctgtcgcccaggctggagtgcagtggcacaatctcagctcactgcaacctctgcctcccgggttcaagcgattcttgtgccttagcctcccaagtagctgggattacaggcacctgccaccatgcccggctaataattttttttgtatttttagtagcgatgaggtttccccatgttggccaggctggtctcaaactcctggcctcaagtgatccacccacctaggcctcccaaagtgctgggattacaggcgtgagccactgcacccggcctagttattgtttttaaaatgttagctttgtgataccatcccaaaaagtcatttattgttttttgtttgtttgggtaggagaattcatcaaagtggacattctataaatttttggttaacaaattggctcaagtcacattcttggcccaaagaccatttttggttttactttcacaggaaatacatatgaaaaagttaggtttgtggctgtcaaactgtcagctgtttttaaaatgtaatttttagtaccaccttaatactaccttataaagaatgcagaatatacttttgtatttggctttcttaaagtgaagagataatgctttaaagctaacctgctcacaaatagctgagaaatttaaaaggagattttacttaacattaactttttttaagctaaaagctcataattttaacatttggcttttctactaccctactgctgaacagagcaataaaaaaaactatactattttatttggacaatactaatataaatccttaacctataatggaaacttccaaacatgaactctaaaacatgggcatttttaatgactaccacttttaataaatatactaaaatattcaatatttgcacatcattaaataaaaaattaatttttaacaaaattttatttagagcattaggaaaatcatattcaaaacacagaaataatcagactataacaatgctgcatagatagtggtatacaagttccctgactctaacttcttcctaacttaaaagttcaattttcaagtcaccaggtagaaaatggtggaggcattatttcctctttctgaggctataaaaaaatggcttcaatggtgagaaggcaaaccatttaaacaatgaagattagattataccccaatttaattctattcccttcttgtttgttatttctcatagatgaaaatttagaatgtaataattattggaaaggaataagaagtgaattacctcttaggagataccctgatcagtgcctgctttaatcagacaaaacactaagttttaaaaattacaaccacaatattatgcctaactaaaattgccaatatgaatacttttttacagaatacattacatgtataccagaagagaaatacttgtttcctatcctctgaccttcagtagaaaaaaaatgttatcactaacaaggatcagaaaaataattttcaaggcagagcattaactcaatggggatcaaaatcttttctgaatacttaaaatagactgagtcagtcaacgagaaattgctaaatttcttctatgagagtacttttcaaaaaggaagacaatttattggaagaatttgtagctggaaacactgttcattaagaaaacattaagttaccctgagaaagactcttaatattaccagtgttttcagggccccctgaccaacgcatggaagagcaacttgtaggctctagccttttaacaatacctacataaagaatattttgatctaaaatgtaacttgggttctctgccacactggtaataagtcacaaccaagacatctgaatgtgatggagtataagcaaattttgcgtttattttaggctgccctctttcttttctaagagaaagagtttgcagttcttcaaatggtcttggatgaaacctactgtttggaaaaaagaatcttctgtaagtaaactggtagttttcttaaaacagtaaacaaatttatctggtctacattctctaaactattattatatgcctagaaaataaggcattagtaattcatcattgaccattgcagagcatagacaactgtttctttctaatcaggaccataagcaaacattcctgaaagtgcagtgttatttttaacgtctcttatgcatttacagtaagcatttgactccctacatactttcattataaaatgttttttcccaacgccttatatataccataattacttaagaaaagacaaagtgagagcagctacagaagtagcaaggtattttccacaaataaaaatacagcatacaaaaaatggcaagttagtgataattggtagtatgagtgcttattaatatcccgctttggggtccaaattaagatttgacaagtttgaagccttgtcctgtgtccagcacagtaggaagaaaccaactcatttttaatcttttcaagcacctaaaacaagttttgcagatccaaaaaaggttcagaccgcataaccaatttgccaaatgcactaggggatatgtaatacgaggaaagtgtaacatccagtgcttggccacatcgcttcccgttggcaaatgcagagtgtagtcactccaccgttttgacacaccatatactgctttcactgtgcgtcccttttcagtccagcagatgttattactggagttgcagttatattctacccagtcttttgtaaagtcacctagctgtggcgggtcagcttcttcaatatctactgtttttatcaactctgctccttgcactgcaatatactggtcattaattttcctcacttctttcacccaaggggttgaattttcgctgtctaatacgataataagccgggaacaaaaggaaccattcttttctctccaccattctataagtgtgtcaaggcgtagtgtatctccacctgctagagcccactctcctgtaccatgggtgtgcccactgtaatacaaaatatacgtatcatgtctgggtccatccactgtccgaagttcgaggaaagcttttagtttggaatgcagagtatcaaatgacagtccacttgtggaatagtcacatccataggtctcaatcatatgatatgcaaaaaatctttggatagcattgagcatgccagtagacctcaaatttaactcctgtacatgttctgggggaagcagtgttggctgaccatcaggactgcagaagttggtgggaatcacaatagcatatccaacagatgttcctcctaaacagttacccaattcatggaagagcccatgagccatggattccaatggcaaaacgattagaaacatgctcaagaaaattccatttgttggctgccaggaaactgctcccaaaatcgctgttgcaagaagactaaagaacaccaactgctctgaaatcaagcaaaaatggcgcatccctttggatgccatgattctatcaaggctattgtaatctgtcctgtgagtaaaatatactttatggcagtcatttaatttggtatggaatccccaaagagttaaaagaaaaataatatgacaaatcatccagaaaattccaaaaatggaaaagccaggtattacaaaataccagaggtgagtgtctctaagtttgaatgcggaaagaataaaaaatgtaagctcaatcattccagcaaaaacgactgaaagtcttctgcaaattcttccacggtacaaaaagggtttccatctttcagttactgaaagtccactaaaataaatgtcaaggaaaggatcagttatcaggcaaataaaaaaacacgcaaaagcaatcggatttttgggagtttccaatgaggaaaaaaataacaaaactgcaaaaataactaagtttggaatagctaagaaagatttcattctcagatcaataatcagcatagccagagctacaacaagcaaaatgacactcagagacttctccaccaacatagttgtgctggcaatggcaaatccaacaagctccagaaattcaactgtggttagtaaagtgggccgatgacggacataaccagaaattctctccaccagagagcacaatatccttaacactatggatgttagaagcaaatatttggttgattcttcttttacatcatttttaaaggatgaattatcaagaaaacataggaggccaagcaagaatccaaaccaaagattggagagacttaaacttgctgcttccattgaaaaatagtaatagagtatgctggcgattccaagaacaaaaagaccaagaataaaaattaccaaaattaaggaatttgctgttttttcccatcttacgtatagacctaagcatatagcaaccaataaattgattctggctaaatagccaagataccgcactgaagaatgcatgttcacttctctatttacttcttccagtcttgtcattgctaaatagagacaatgactaaagcaataacgcagtgatttacacatgtaaccagcaatgtgggcttttccctcacgttacaaaaattaaccgcttgtatttcatccagtatatccaatgtatccgcaactcctatttcaacattttctcttgtggaaattttgtttatagtgatctgactcggccgtcgccaccaacgcgctctcccaaccctcggagtcagttccaaaaccaaaccaaaaaggaggagagcagacaaggcttcagcctgcgactgagaacagggaggcggcacgccttggggaacgagggcccgaggccatacgcgctaatacaggccagtgtcggcgtaaactttctccgttaccggcccggccgcgaccgccatgtttccgccgccgaaatccgc

SEQ ID NO: 13853 - RNA, 4981 nt, Homo sapiens
  source 1..4981: mol_type = other RNA
gctgggattacaggcatgagccaccatgcctggctaaacatgtacttttttttttttttgagacaaagaaagagtcctgctctgtcgcccaggctggagtgcagtggcacaatctcagctcactgcaacctctgcctcccgggttcaagcgattcttgtgccttagcctcccaagtagctgggattacaggcacctgccaccatgcccggctaataattttttttgtatttttagtagcgatgaggtttccccatgttggccaggctggtctcaaactcctggcctcaagtgatccacccacctaggcctcccaaagtgctgggattacaggcgtgagccactgcacccggcctagttattgtttttaaaatgttagctttgtgataccatcccaaaaagtcatttattgttttttgtttgtttgggtaggagaattcatcaaagtggacattctataaatttttggttaacaaattggctcaagtcacattcttggcccaaagaccatttttggttttactttcacaggaaatacatatgaaaaagttaggtttgtggctgtcaaactgtcagctgtttttaaaatgtaatttttagtaccaccttaatactaccttataaagaatgcagaatatacttttgtatttggctttcttaaagtgaagagataatgctttaaagctaacctgctcacaaatagctgagaaatttaaaaggagattttacttaacattaactttttttaagctaaaagctcataattttaacatttggcttttctactaccctactgctgaacagagcaataaaaaaaactatactattttatttggacaatactaatataaatccttaacctataatggaaacttccaaacatgaactctaaaacatgggcatttttaatgactaccacttttaataaatatactaaaatattcaatatttgcacatcattaaataaaaaattaatttttaacaaaattttatttagagcattaggaaaatcatattcaaaacacagaaataatcagactataacaatgctgcatagatagtggtatacaagttccctgactctaacttcttcctaacttaaaagttcaattttcaagtcaccaggtagaaaatggtggaggcattatttcctctttctgaggctataaaaaaatggcttcaatggtgagaaggcaaaccatttaaacaatgaagattagattataccccaatttaattctattcccttcttgtttgttatttctcatagatgaaaatttagaatgtaataattattggaaaggaataagaagtgaattacctcttaggagataccctgatcagtgcctgctttaatcagacaaaacactaagttttaaaaattacaaccacaatattatgcctaactaaaattgccaatatgaatacttttttacagaatacattacatgtataccagaagagaaatacttgtttcctatcctctgaccttcagtagaaaaaaaatgttatcactaacaaggatcagaaaaataattttcaaggcagagcattaactcaatggggatcaaaatcttttctgaatacttaaaatagactgagtcagtcaacgagaaattgctaaatttcttctatgagagtacttttcaaaaaggaagacaatttattggaagaatttgtagctggaaacactgttcattaagaaaacattaagttaccctgagaaagactcttaatattaccagtgttttcagggccccctgaccaacgcatggaagagcaacttgtaggctctagccttttaacaatacctacataaagaatattttgatctaaaatgtaacttgggttctctgccacactggtaataagtcacaaccaagacatctgaatgtgatggagtataagcaaattttgcgtttattttaggctgccctctttcttttctaagagaaagagtttgcagttcttcaaatggtcttggatgaaacctactgtttggaaaaaagaatcttctgtaagtaaactggtagttttcttaaaacagtaaacaaatttatctggtctacattctctaaactattattatatgcctagaaaataaggcattagtaattcatcattgaccattgcagagcatagacaactgtttctttctaatcaggaccataagcaaacattcctgaaagtgcagtgttatttttaacgtctcttatgcatttacagtaagcatttgactccctacatactttcattataaaatgttttttcccaacgccttatatataccataattacttaagaaaagacaaagtgagagcagctacagaagtagcaaggtattttccacaaataaaaatacagcatacaaaaaatggcaagttagtgataattggtagtatgagtgcttattaatatcccgctttggggtccaaattaagatttgacaagtttgaagccttgtcctgtgtccagcacagtaggaagaaaccaactcatttttaatcttttcaagcacctaaaacaagttttgcagatccaaaaaaggttcagaccgcataaccaatttgccaaatgcactaggggatatgtaatacgaggaaagtgtaacatccagtgcttggccacatcgcttcccgttggcaaatgcagagtgtagtcactccaccgttttgacacaccatatactgctttcactgtgcgtcccttttcagtccagcagatgttattactggagttgcagttatattctacccagtcttttgtaaagtcacctagctgtggcgggtcagcttcttcaatatctactgtttttatcaactctgctccttgcactgcaatatactggtcattaattttcctcacttctttcacccaaggggttgaattttcgctgtctaatacgataataagccgggaacaaaaggaaccattcttttctctccaccattctataagtgtgtcaaggcgtagtgtatctccacctgctagagcccactctcctgtaccatgggtgtgcccactgtaatacaaaatatacgtatcatgtctgggtccatccactgtccgaagttcgaggaaagcttttagtttggaatgcagagtatcaaatgacagtccacttgtggaatagtcacatccataggtctcaatcatatgatatgcaaaaaatctttggatagcattgagcatgccagtagacctcaaatttaactcctgtacatgttctgggggaagcagtgttggctgaccatcaggactgcagaagttggtgggaatcacaatagcatatccaacagatgttcctcctaaacagttacccaattcatggaagagcccatgagccatggattccaatggcaaaacgattagaaacatgctcaagaaaattccatttgttggctgccaggaaactgctcccaaaatcgctgttgcaagaagactaaagaacaccaactgctctgaaatcaagcaaaaatggcgcatccctttggatgccatgattctatcaaggctattgtaatctgtcctgtgagtaaaatatactttatggcagtcatttaatttggtatggaatccccaaagagttaaaagaaaaataatatgacaaatcatccagaaaattccaaaaatggaaaagccaggtattacaaaataccagaggtgagtgtctctaagtttgaatgcggaaagaataaaaaatgtaagctcaatcattccagcaaaaacgactgaaagtcttctgcaaattcttccacggtacaaaaagggtttccatctttcagttactgaaagtccactaaaataaatgtcaaggaaaggatcagttatcaggcaaataaaaaaacacgcaaaagcaatcggatttttgggagtttccaatgaggaaaaaaataacaaaactgcaaaaataactaagtttggaatagctaagaaagatttcattctcagatcaataatcagcatagccagagctacaacaagcaaaatgacactcagagacttctccaccaacatagttgtgctggcaatggcaaatccaacaagctccagaaattcaactgtggttagtaaagtgggccgatgacggacataaccagaaattctctccaccagagagcacaatatccttaacactatggatgttagaagcaaatatttggttgattcttcttttacatcatttttaaaggatgaattatcaagaaaacataggaggccaagcaagaatccaaaccaaagattggagagacttaaacttgctgcttccattgaaaaatagtaatagagtatgctggcgattccaagaacaaaaagaccaagaataaaaattaccaaaattaaggaatttgctgttttttcccatcttacgtatagacctaagcatatagcaaccaataaattgattctggctaaatagccaagataccgcactgaagaatgcatgttcacttctctatttacttcttccagtcttgtcattgctaaatagagacaatgactaaagcaataacgcagtgatttacacatgtaaccagcaatgtgggcttttccctcacgttacaaaaattaaccgcttgtatttcatccagtatatccaatgtatccgcaactcctatttcaacattttctcttgtggaaattttgtttatagtgatcttcctatggaccaaaatcaacatggcagattgtttttaaatggctaatttacaaaactcttccccattctgatcttcttcaaaagacagcctgactcggccgtcgccaccaacgcgctctcccaaccctcggagtcagttccaaaaccaaaccaaaaaggaggagagcagacaaggcttcagcctgcgactgagaacagggaggcggcacgccttggggaacgagggcccgaggccatacgcgctaatacaggccagtgtcggcgtaaactttctccgttaccggcccggccgcgaccgccatgtttccgccgccgaaatccgc

SEQ ID NO: 13854 - RNA, 2782 nt, Homo sapiens
  source 1..2782: mol_type = other RNA
gctgggattacaggcatgagccaccatgcctggctaattttgtatttttaatagagacagcatttcaccatcttggtcaggctggtcttgaactcctgacctcaaatgatccacctgccttggcctcccaaagtgctgggattacaggcgtgagccaccatgcccggccatttgttattgttatgattgtcttggctctccaactaaaggataagttctttgaagttgacacataatagttttcaataaatggtagctatgatgatgatgatgatgatgatgataatgatgatagctatgatgatgatgatgatgacgatgatgatgatgatgacaatggtgatgatgacgatgacgatggtgacgttgatgtatacagttcaggctcttgttgtattttgtggttgtttttaaaccaagtgatctgaggctcggggacaccattagcatgacagtctaaagtggtggaactgctgatggccactgtgtgatcactgaggtttcgcaggaggtatggtgcttcctgatctctgattgtaatttctttcttctggaggatttcttcccctgtgtatacattcctggctctgcaggcataggtgcctgaatcttgcagggaaacattcatgatggtaagattaagagtgatggagtgctccttagtgatggccattttttgcttgctaatactgtagtgcattgttctgttattaactgtccgcagtaaaatccaagtaacgtctctgtataagaacttgttaactgtgcaagacagtttcaggtcctctccttccgtcggcattttttccaagttaacatgaaacccatttggcacatctgtgatataaaagcttatgtttcttcccacagtcccaactttattggaagctatgcaaatgtagattccagaaattctagagtcagccacaaccaaggtgctagccatcttattctttccttctattattgccatgcgctgagtgatgctctcaattctgtttcccatgttgctgtcagcatccaggataaaggactcttcattattggaacaaaagtcacaccttgcttcggaatgattatggttacaggggtgccagaaccacttgattgtaggttgagggataccatatgcggtacaagtcaggatttgtctgctgcccagtgggtagagagccgggtctggaaacgatgacacggccttttcgtaaatctggggtttcacattgacaattagagtggcagtgaggtttttaaacacatttgactgttttatgctcagcaagattgtataattccctgcatcctcttcagttacgtccttgataattaacgagtagccacgagtcaaatagcgagcagatttctcagtcgcaggtaacccatcttttaaccatacaacttccggcgagggaaatgccttcactttcatagagagccggtaagaccgcttgccagctacggtttcaagcacctgctgttttcgatgtttcacagtgatgaatgctttatcatatatatgcactgaggtgttaacagatttgaatgatggtccactccttacacgacaagtataaagtcctttgtctttgttctgcattttgtcaatagtaagaacactgtagaatatgttggcatgggaattgctttggtcaattcgtcgccttacggaagctctcttatttttttcatcagggtaactccaggtcatttgaactctcgtgttcaagggagtggtagcagtacaattgaggacaagagtatggcctctaagtaatttgactgggcgtggtgtgcttatttggacatctatgattgtattggtttgtcgatgtgtgagatagtttgtcttatacaaatgcccattgactgttgcttcacaggtcagaagccctatttctttgtacgttgcatttgatatgatgaagccctttctactgtcccagattatgcgttttccatcagggatcaaagtgtcaagtggaaacttttttaaagtaacagtgatgttaggtgacgtaacccggcagggaatgacgagctcccttccttcagtcatgtgtataatttcggggatttcactgtacatctctacgaaaggtctacctgtatcactaataaatatatagattgcagattctgtttccttcttctttgaagtaggtacagctagatatttgcagctgtagaagccagtgtggtttgcttgagctgtgttcaaggttaaagtactgcagaattgtttgccatttcttccacaggcagatttagttatgctcagcctttcgctttccttactcaccatttcaggcaaagaccatttatgggctgcttcccccctgcattggagatgcagtgtctggcctgcttgcatgatgtgctgggtgccttttaaactcagttcaggatcttttaattttgaacctgaactagatcctgtgagaagcagacagctgagcagcgcgcacagcaggaccccggtgtcccagtagctgaccatggtgagcgcgacgcggcctgctcgcccggtgcccgcgctccccgcggccaacgacccggccgccagagtccgtcctctcgttcgccgccgccggccccgcgccctgagcgcccgtctcgcggctccagccaggagacaaccacttccccgggtaatcctcgccgccaggcgcccgctggccgctgcacccgagccccggagcccgctccgagccgccgccgctgccggggaggagccgagaggagtgtccgcctggcgcgctccgagcctcccgcggacctcgat

SEQ ID NO: 13855 - RNA, 1529 nt, Homo sapiens
  source 1..1529: mol_type = other RNA
gctgggattacaggcatgagccaccatgcctggctattaaccttgtttctaacttcagcattgcacatctccttagtaaagcagtagccattaacaagtcaggtccaacaaccattttcctctggtcctcaagcagagactcagagccagttacacataaactatttcattataacatgaaaatagcaagccttgggctattgcaaaaggcttttcaaatgttgacctctaacttggagaaaatagagggaagcagaaatatagggtgctaatttgtgctataacctggtctcatgtcgtggtatattcccagttgcaacattttaaatttataagtgagaaagtaaaacaaagcttcatatctgtgaaagtgaaaaattgtccagaagtcttctattcaaagaccaattagctttttcttcccaataacttatcagaaagaaatgggtacttagaaacctaaggggttctttaaataggagtcagaaaaaatatataaaaataaaaaacaaagcaagaaagaacattgtataaaaataaaatgttctttaaagatgactgccctctcttgaaagatgagtgctatattaaaagggtagatgtatctctataactcatcgtgtttatatgtaaattctctggcagatataaacccatctttgtcttcatcttctttatcaaaaatatcctccaccaaagcatcatgatgactttcattcaccaccgcaccatgtttttcaaactccttctttaaatatgctttaacctcatctttagagagtttccagtcatcattaagatccatttcttggaatgattcatgggatcttggtccatttcgaatctccaggagatcaatattaaatatcagtgtactttctgggggaattttaccatttcagatctagacagagatgtgacatgcgctaggttgttgataaaactggtatctttccaaaagaggcatgcaagcatgtactaaaagacttttccttcttttccatagcccagagcaggaggaatgatgagctttctcttctctcctacacacattcctttcaagccctggtcccaacctttgagagcctccaggatgcccagggtaaaccaaatgggctgaccattgttatgtttgtgagtggagtgaaataaggagccgtccttttctaagtagccttcatagtggaccaacatcaaatcccctcctttggtcttgcgatggcagatgaatggcttctggagaacttcaattttcacttctggttcagggatcaaagccccaatcaaagaagtgacgaacagagtcaagaccgcgttccacaagaaaagcctcatgttgctgaagcaaggaaagaagtccctacaaaagcagcgaaaggtccctcgacttcatagatttaagaacgtagttcaaggcttacggacaagggcttcagacaagttcaggactcccccttcttagaagacgtggcacatttaccaccaactcttttctcaagggtcacgaacctacctttaaagagttaagc

SEQ ID NO: 13856 - RNA, 1437 nt, Homo sapiens
  source 1..1437: mol_type = other RNA
gctgggattacaggcatgagccaccatgcctggctattaaccttgtttctaacttcagcattgcacatctccttagtaaagcagtagccattaacaagtcaggtccaacaaccattttcctctggtcctcaagcagagactcagagccagttacacataaactatttcattataacatgaaaatagcaagccttgggctattgcaaaaggcttttcaaatgttgacctctaacttggagaaaatagagggaagcagaaatatagggtgctaatttgtgctataacctggtctcatgtcgtggtatattcccagttgcaacattttaaatttataagtgagaaagtaaaacaaagcttcatatctgtgaaagtgaaaaattgtccagaagtcttctattcaaagaccaattagctttttcttcccaataacttatcagaaagaaatgggtacttagaaacctaaggggttctttaaataggagtcagaaaaaatatataaaaataaaaaacaaagcaagaaagaacattgtataaaaataaaatgttctttaaagatgactgccctctcttgaaagatgagtgctatattaaaagggtagatgtatctctataactcatcgtgtttatatgtaaattctctggcagatataaacccatctttgtcttcatcttctttatcaaaaatatcctccaccaaagcatcatgatgactttcattcaccaccgcaccatgtttttcaaactccttctttaaatatgctttaacctcatctttagagagtttccagtcatcattaagatccatttcttggaatgattcatgggatcttggtccatttcgaatctccaggagatcaatattaaatatcagtgtactttctgggggaattttaccttttccttcttttccatagcccagagcaggaggaatgatgagctttctcttctctcctacacacattcctttcaagccctggtcccaacctttgagagcctccaggatgcccagggtaaaccaaatgggctgaccattgttatgtttgtgagtggagtgaaataaggagccgtccttttctaagtagccttcatagtggaccaacatcaaatcccctcctttggtcttgcgatggcagatgaatggcttctggagaacttcaattttcacttctggttcagggatcaaagccccaatcaaagaagtgacgaacagagtcaagaccgcgttccacaagaaaagcctcatgttgctgaagcaaggaaagaagtccctacaaaagcagcgaaaggtccctcgacttcatagatttaagaacgtagttcaaggcttacggacaagggcttcagacaagttcaggactcccccttcttagaagacgtggcacatttaccaccaactcttttctcaagggtcacgaacctacctttaaagagttaagc

SEQ ID NO: 13857 - RNA, 1285 nt, Homo sapiens
  source 1..1285: mol_type = other RNA
gctgggattacaggcatgagccaccatgcctggctattaaccttgtttctaacttcagcattgcacatctccttagtaaagcagtagccattaacaagtcaggtccaacaaccattttcctctggtcctcaagcagagactcagagccagttacacataaactatttcattataacatgaaaatagcaagccttgggctattgcaaaaggcttttcaaatgttgacctctaacttggagaaaatagagggaagcagaaatatagggtgctaatttgtgctataacctggtctcatgtcgtggtatattcccagttgcaacattttaaatttataagtgagaaagtaaaacaaagcttcatatctgtgaaagtgaaaaattgtccagaagtcttctattcaaagaccaattagctttttcttcccaataacttatcagaaagaaatgggtacttagaaacctaaggggttctttaaataggagtcagaaaaaatatataaaaataaaaaacaaagcaagaaagaacattgtataaaaataaaatgttctttaaagatgactgccctctcttgaaagatgagtgctatattaaaagggtagatgtatctctataactcatcgtgtttatatgtaaattctctggcagatataaacccatctttgtcttcatcttctttatcaaaaatatcctccaccaaagcatcatgatgactttcattcaccaccgcaccatgtttttcaaactccttctttaaatatgctttaacctcatctttagagagtttccagtcatcattaagatccatttcttggaatgattcatgggatcttggtccatttcgaatctccaggagatcaatattaaatatcagtgtactttctgggggaattttacgtggagtgaaataaggagccgtccttttctaagtagccttcatagtggaccaacatcaaatcccctcctttggtcttgcgatggcagatgaatggcttctggagaacttcaattttcacttctggttcagggatcaaagccccaatcaaagaagtgacgaacagagtcaagaccgcgttccacaagaaaagcctcatgttgctgaagcaaggaaagaagtccctacaaaagcagcgaaaggtccctcgacttcatagatttaagaacgtagttcaaggcttacggacaagggcttcagacaagttcaggactcccccttcttagaagacgtggcacatttaccaccaactcttttctcaagggtcacgaacctacctttaaagagttaagc

SEQ ID NO: 13858 - RNA, 2689 nt, Homo sapiens
  source 1..2689: mol_type = other RNA
gctgggattacaggcatgagccaccatgcctggctggctttccctcttgagcacatgcatgtaggcaggaatcccagccccctttgcagatgagcaaactgagacacagagaggttcagccacctgcgaaggttgcacagccaggatccaccgccttctcgcagcacccaccctcttcccaaggagtgcccagttcagcaaggcagatgacaccaatcccaactgggcagccaggttttatgaggccaggacaaacagcactgatttgaagccttgtagaggggttcaaatcacaggccctgccacaggctggcctcagggtcctgggggagctgtgggcatgcttctgagccgtagctcctctatccacccaagggagctggtagcactggccttaagagtgtgctgtgagcccggggggttgcagctgggcattgaatgattcctaccaccccacaaataccactctgcccctccaacgggggcaacccctcatggcctgtctcggcagcatggaagttacactctattgcatcacccccaggaagatggagagaggcctccaggacctcatgagggtggttttctgcataatgagatgccttggatattcctagaggtccgagcctaggcctctgtcagcacatcagtgaatgcagccctgctggacaagctcaggaggactccaggatcccgagtgacacattccacatccatacaggcagaccagggcctgcaattacagatgggaggtcccaaggtccaggcaggggctcccacatgttcccaggaaagcaccaggcagggagggtggtgggcagcagttctgggctttgctcctcgccaggccccatttcttcatctgtaaaatggggagaaaatattttcccttcctaactgcattggaaagacgagataagcagccgactggggaaggtggaacttcccactcaagcaatattgggcgaaataagtgggttcagagactgagcggtggtgctggccccagacactggtgtggatgcaacacgtcgcaggactcagcccgtcgaacccctgcctgccgctgcactgatgcccccttccccctcacagagccctgatgcccggccatcctgatggcgggagctcccctaggcctctacagccgtggtccaaacgaaccctgcactccacaccggggctcctcaccactggggcaccctgggctgccctcggggctggcactcggtggtgggggccgtccgacacctggtaggatgctgagccgcacccccggcctccacccactagacgttggtagcattcattgtgacaacaaatttatacctaaacattgccaatactgcccccagtggagaaccaatgacgggtagtctagactgtccatgtcaccttctcttagtccttccccggactgggacgtctcacaaccaagtccttgtcccaccccactctctacatcccggcatccagcaccgccccctgctgagggctcggccaatgtttcctgaatgaatgagtggcccctggatgtgagcatgggtcacacacctcacggtgattgggtgggggtttctcatgagtagagggacccccacatgccagggctgcgctgagcagggacgtcagtgactccctctgtgaaggcggccacttgagacaggattctaggagcctctgtcacacccggcagtgcacaggatgattcagagagaggctgtcccaaggcctcccggctcactggtcgcagtcttccaggtcctcccgccaccctccacacagcaccactgccaccctcatccctgctgggcaggagaggcggtcgggagggcagacacagggcagtgggcgagtctgatccgggttttgtgaggcctccaaaatccagaaaaccaacatcgtgtttttacgaagggcctgctccatctccataacacttcttcttgaactttttggctgcgtactttttatctatctcattgtttgagaattttacatcaccccagccggatgtcccaccacactcctgcctgggaacttctggcacgcaggagaggctggacacgcagatgcagagaggcttgccccaacgccgttgcccgttttaccttgaagttcgtggttctttaattcttgctccaaactgtgaatcaacctttaaaatatatgatattgaagttctccttcagcctccagtctttcatcagagttaaatccagagatttcacgagcagtagataaatttgcagtagagaaaagtgctccaaaggtgggcacgcctggctcccatttggaggtgtttataaatgcttttatgtagacccctcctagatgacaaggaatggcctcagagcaaccctgggaaggatgaggaggggtctggggactccagacgaaattgcacagccgcctaccgtgtgagtggaaacccatgctgcttctgcctggcctctaggatccgcgttcaggggaagccgtgtccctgagtctctcctaggcctgttctggatccgaagtgggtatgagacattcaccatctattcctttgctccaccgtcaccagaggctttgtggtaccttatttttgagaagaggcaacatattctaggactaggctgggaacaagggagaaattcatcatgcatccctccatttatccatccatccatccatccatccatccatc

SEQ ID NO: 13859 - RNA, 3198 nt, Homo sapiens
  source 1..3198: mol_type = other RNA
gctgggattacaggcatgagccaccatgcctggctggctttccctcttgagcacatgcatgtaggcaggaatcccagccccctttgcagatgagcaaactgagacacagagaggttcagccacctgcgaaggttgcacagccaggatccaccgccttctcgcagcacccaccctcttcccaaggagtgcccagttcagcaaggcagatgacaccaatcccaactgggcagccaggttttatgaggccaggacaaacagcactgatttgaagccttgtagaggggttcaaatcacaggccctgccacaggctggcctcagggtcctgggggagctgtgggcatgcttctgagccgtagctcctctatccacccaagggagctggtagcactggccttaagagtgtgctgtgagcccggggggttgcagctgggcattgaatgattcctaccaccccacaaataccactctgcccctccaacgggggcaacccctcatggcctgtctcggcagcatggaagttacactctattgcatcacccccaggaagatggagagaggcctccaggacctcatgagggtggttttctgcataatgagatgccttggatattcctagaggtccgagcctaggcctctgtcagcacatcagtgaatgcagccctgctggacaagctcaggaggactccaggatcccgagtgacacattccacatccatacaggcagaccagggcctgcaattacagatgggaggtcccaaggtccaggcaggggctcccacatgttcccaggaaagcaccaggcagggagggtggtgggcagcagttctgggctttgctcctcgccaggccccatttcttcatctgtaaaatggggagaaaatattttcccttcctaactgcattggaaagacgagataagcagccgactggggaaggtggaacttcccactcaagcaatattgggcgaaataagtgggttcagagactgagcggtggtgctggccccagacactggtgtggatgcaacacgtcgcaggactcagcccgtcgaacccctgcctgccgctgcactgatgcccccttccccctcacagagccctgatgcccggccatcctgatggcgggagctcccctaggcctctacagccgtggtccaaacgaaccctgcactccacaccggggctcctcaccactggggcaccctgggctgccctcggggctggcactcggtggtgggggccgtccgacacctggtaggatgctgagccgcacccccggcctccacccactagacgttggtagcattcattgtgacaacaaatttatacctaaacattgccaatactgcccccagtggagaaccaatgacgggtagtctagactgtccatgtcaccttctcttagtccttccccggactgggacgtctcacaaccaagtccttgtcccaccccactctctacatcccggcatccagcaccgccccctgctgagggctcggccaatgtttcctgaatgaatgagtggcccctggatgtgagcatgggtcacacacctcacggtgattgggtgggggtttctcatgagtagagggacccccacatgccagggctgcgctgagcagggacgtcagtgactccctctgtgaaggcggccacttgagacaggattctaggagcctctgtcacacccggcagtgcacaggatgattcagagagaggctgtcccaaggcctcccggctcactggtcgcagtcttccaggtcctcccgccaccctccacacagcaccactgccaccctcatccctgctgggcaggagaggcggtcgggagggcagacacagggcagtgggcgagtctgatccgggttttgtgaggcctccaaaatccagaaaaccaacatcgtgtttttacgaagggcctgctccatctccataacacttcttcttgaactttttggctgcgtactttttatctatctcattgtttgagaattttacatcaccccagccggatgtcccaccacactcctgcctgggaacttctggcacgcaggagaggctggacacgcagatgcagagaggcttgccccaacgccgttgcccgttttaccttgaagttcgtggttctttaattcttgctccaaactgtgaatcaacctttaaaatatatgatattgaagttctccttcagcctccagtctttcatcagagttaaatccagagatttcacgagcagtagataaatttgcagtagagaaaagtgctccaaaggtgggcacgcctggctcccatttggaggtgtttataaatgcttttatgtagacccctcctagatgacaaggaatggcctcagagcaaccctgggaaggatgaggaggggtctggggactccagacgaaattgcacagccgcctaccgtgtgagtggaaacccatgctgcttctgcctggcctctaggatccgcgttcaggggaagccgtgtccctgcggtcatgagacgtgattgttcagaccaatggatgaggctgagcagaatcatttcatttcccccgcacttgccaaaggcagggactttcctgtttgtccctgcctgatatgcaggaagggctcagaactacttaagaacaaatcaatgaacctatggctttatggcaaataccacagaaacaaccttagaaatgggctgaggaggctgtctggcctctaacaaatgacctcatctctctgaaccttaacttcctcatcagtaaagtggcagtgcagcccctccctcacaggacgctccctggcagagtgcagccctgccgtgcagcagccggtatgacctcgtccttgtgatcaggagggccctgctgaactgtttccgccccgcaggtgcctacgaagcctgggaaatgatgtggccttcctggagccatgcaatggctttgttgtcaccaggaaaagggcctgtggcacccgcctggccactcatgtcctaaatgagacaggccctcttcatcggcctcagtggctcattgagatgaggacttgggaattttgctgtttaacagagcaactgagcacccaggtggctgccccagcagaccctggagacgtttcaggagacctggcagggacccaagcctctgccactgcaccaggccctggccagagggctgggctcagagccctttatttttttatttttatttttt

SEQ ID NO: 13860 - RNA, 3655 nt, Homo sapiens
  source 1..3655: mol_type = other RNA
gctgggattacaggcatgagccaccatgcctggctggctttccctcttgagcacatgcatgtaggcaggaatcccagccccctttgcagatgagcaaactgagacacagagaggttcagccacctgcgaaggttgcacagccaggatccaccgccttctcgcagcacccaccctcttcccaaggagtgcccagttcagcaaggcagatgacaccaatcccaactgggcagccaggttttatgaggccaggacaaacagcactgatttgaagccttgtagaggggttcaaatcacaggccctgccacaggctggcctcagggtcctgggggagctgtgggcatgcttctgagccgtagctcctctatccacccaagggagctggtagcactggccttaagagtgtgctgtgagcccggggggttgcagctgggcattgaatgattcctaccaccccacaaataccactctgcccctccaacgggggcaacccctcatggcctgtctcggcagcgtggaagttacactctattgcatcacccccaggaagatggagagaggcccccaggacctcatgagggtggttttctgcgtaatgagatgctttggatattcctagaggtccgagcctaggcctctgtcagcacatcagtgaatgcagccctgctggacaagctcaggaggactccaggatcccgagtgacacattccaaatccacacaggcagaccggggcctgcaattacagatgggaggtcccaaggtccaggcaggggctcccacatgttcccaggaaagcaccaggcagggagggtggtgggcagcagttctgggctttgctcctcgccaggccccatttcttcatctcacggtgattgggtgggggtttctcatgagtagagggacccccacatgccagggctgcgctgagcagggacgtcagtgactccctctgtgaaggcggccacttgagacaggattctaggagcctctgtcacacccggcagtgcacaggatgattcagagagaggctgtcccaaggcctcccggctcactggtcgcagtcttccaggtcctcccgccaccctccacacagcaccactgccaccctcatccctgctgggcaggagaggcggtcgggagggcagacacagggcagtgggcgagtctgatccgggttttgtgaggcctccaaaatccagaaaaccaacatcgtgtttttacgaagggcctgctccatctccataacacttcttcttgaactttttggctgcgtactttttatctatctcattgtttgagaattttacatcaccccagccggatgtcccaccacactcctgcctggggacttctggcatgcaggagaggctggacacgcagatgcagagaggcttgccccaacgccgttgcccgttttaccttgaagttcgtggttctttaattcttgctccaaactgtgaatcaacctttaaaatatatgatattgaagttctccttcagcctccagtctttcatcagagttaaatccagagatttcacgagcagtagataaatttgcagtagagaaaagtgctccaaaggtgggcacgcctggctcccatttggaggtgtttataaatgcttttatgtagacccctcctagatgacgaggaatggcctcagagcaaccctgggaaggatgaggaggggtctgcggactccagacgaaattgcacagccgcctaccgtgtgagtggaaacccatgctgcttctgcctggcctctaggatccgcgttcaggggaagccgtgtccctgcggtcatgagacgtgattgttcagaccaatggatgaggctgagcagaatcatttcatttcccccgcacttgccaaaggcagggactttcctgtttgtccctgcctgatatgcaggaagggctcagaactacttaagaacaaatcaatgaacctatggctttatggcaaataccacagaaacaaccttagaaatgggctgaggaggctgtctggcctctaacaaatgacctcatctctctgaaccttaatttcctcatcagtaaagtggcagtgcagcccctccctcacaggacgctccctggcagagtgcagccctgccgtgcagcagccggtatgacctcttccttgtgatcaggagggccctgctgaactgtttccgccccgcaggtgcctacgaagcccgggaaatgatgtggccttcctggagccatgcaatggctttgttgtcaccaggaaaagggcctgtggcacccgcctggccactcatgtcctaaatgagacaggccctcttcatcggcctcagtggctcattgagatgaggacttgggaattttgctgtttaacagagcaactgagcacccaggtggctgccccagcagaccctggagacgtttcaggagacctggcagggacccaagcctctgccactgcaccaggccctggccagagggctgggctcagagccctttatttttttatttttattttttattttttagagacacagtattgccctgtctcccaggctggagcacagcagttgaaaccatacctcactgcagcctcgatctcccaggcttaaatgattctcctgcctcagcctccaagtagctgggaccacaggcatatgccaccatgccagccttattgttaaatgttttgggtagatcccatctccctatgttgctcaggctggtcttgaactcctgggctcaagcgttcctcacatctcagcctcttgagtagctgagaccacaagtgtgtgccaccgcacctggccccagagccccttttaaactgcaactcacagtctccaagttagactcacacagagaagatctaaatatgtgtctccttgagggaggctgaggagtggaggaggatgaactcttacaaaacatcaacctttttaaaaatgtgttttcagtaattgctgttctgcgccaagttttatcctagtgggagtttcatgtcagaattactaagtaggagttcataacagagaagttaatcgcccttgtgtaggggcgaggcaccgagcgatgatctctgtgcccaggtaggtgcttcctggatccgcacaagcacaggagatggcaggtggggagtgggtggggggttatgaagggcagccgaggaggggcagggggcagggggaagcaggatctctgacggtagaagggagtggtcactacgtccccaacacacccccttcatgtccccgctatagccacacaccacgggggaaaggctccaggccagcccccatcccctcaggaccatgatgcgggcatctgcagaaacgggtgggggctgtctggcctgagaggcctagagccaggaacaggtggtttagagctgccctcctcctccaacttcagccccaacccccttcctcagcagcagatcccacctgagtctctcctaggcctgttctggatccgaagtgggtatgagacattcaccatctattcctttgctccaccgtcaccagaggctttgtggtaccttatttttgagaagaggcaacatattctaggactaggctgggaacaagggagaagttcatcatgcatccctccatttatccatccatccatccatccatccatccatcatccattctcccacctacccac

SEQ ID NO: 13861 - RNA, 4347 nt, Homo sapiens
  source 1..4347: mol_type = other RNA
gctgggattacaggcatgagccaccatgcctggctggctttccctcttgagcacatgcatgtaggcaggaatcccagccccctttgcagatgagcaaactgagacacagagaggttcagccacctgcgaaggttgcacagccaggatccaccgccttctcgcagcacccaccctcttcccaaggagtgcccagttcagcaaggcagatgacaccaatcccaactgggcagccaggttttatgaggccaggacaaacagcactgatttgaagccttgtagaggggttcaaatcacaggccctgccacaggctggcctcagggtcctgggggagctgtgggcatgcttctgagccgtagctcctctatccacccaagggagctggtagcactggccttaagagtgtgctgtgagcccggggggttgcagctgggcattgaatgattcctaccaccccacaaataccactctgcccctccaacgggggcaacccctcatggcctgtctcggcagcgtggaagttacactctattgcatcacccccaggaagatggagagaggcccccaggacctcatgagggtggttttctgcgtaatgagatgctttggatattcctagaggtccgagcctaggcctctgtcagcacatcagtgaatgcagccctgctggacaagctcaggaggactccaggatcccgagtgacacattccaaatccacacaggcagaccggggcctgcaattacagatgggaggtcccaaggtccaggcaggggctcccacatgttcccaggaaagcaccaggcagggagggtggtgggcagcagttctgggctttgctcctcgccaggccccatttcttcatctgtaaaatggggagaaaatattttcccttcctaactgcattggaaagacgagataagcagccgactggggaaggtggaacttcccactcaagcaatattgggcgaaataagtgggttcagagactgagcggtggtgctggccccagacactggtgtggatgcaacacgtcgcaggactcagcccgtcgaacccctgcctgccgctgcactgatgcccccttccccctcacagagccctgatgcccggccatcctgatggcgggagctcccctaggcctctacagccgtggtccaaacgaaccctgcactccacaccggggctcctcaccactggggcaccctgggctgccctcggggctggcactcggtggtgggggccgtccgacacctggtaggatgctgagccgcacccccggcctccacccactagacgttggtagcattcattgtgacaaccaatttatacctaaacattgccaatactgcccccagtggagaaccaatgactggtagtctagactgtccatgtcaccttctcttagtccttccccggactgggacgtctcacaaccaagtccttgtcccaccccactctctacatcccggcatccagcaccgccccctgctgagggctcggccaatgtttcctgaatgaatgagtggcccctggatgtgagcatgggtcacacacctcacggtgattgggtgggggtttctcatgagtagagggacccccacatgccagggctgcgctgagcagggacgtcagtgactccctctgtgaaggcggccacttgagacaggattctaggagcctctgtcacacccggcagtgcacaggatgattcagagagaggctgtcccaaggcctcccggctcactggtcgcagtcttccaggtcctcccgccaccctccacacagcaccactgccaccctcatccctgctgggcaggagaggcggtcgggagggcagacacagggcagtgggcgagtctgatccgggttttgtgaggcctccaaaatccagaaaaccaacatcgtgtttttacgaagggcctgctccatctccataacacttcttcttgaactttttggctgcgtactttttatctatctcattgtttgagaattttacatcaccccagccggatgtcccaccacactcctgcctggggacttctggcatgcaggagaggctggacacgcagatgcagagaggcttgccccaacgccgttgcccgttttaccttgaagttcgtggttctttaattcttgctccaaactgtgaatcaacctttaaaatatatgatattgaagttctccttcagcctccagtctttcatcagagttaaatccagagatttcacgagcagtagataaatttgcagtagagaaaagtgctccaaaggtgggcacgcctggctcccatttggaggtgtttataaatgcttttatgtagacccctcctagatgacgaggaatggcctcagagcaaccctgggaaggatgaggaggggtctgcggactccagacgaaattgcacagccgcctaccgtgtgagtggaaacccatgctgcttctgcctggcctctaggatccgcgttcaggggaagccgtgtccctgcggtcatgagacgtgattgttcagaccaatggatgaggctgagcagaatcatttcatttcccccgcacttgccaaaggcagggactttcctgtttgtccctgcctgatatgcaggaagggctcagaactacttaagaacaaatcaatgaacctatggctttatggcaaataccacagaaacaaccttagaaatgggctgaggaggctgtctggcctctaacaaatgacctcatctctctgaaccttaatttcctcatcagtaaagtggcagtgcagcccctccctcacaggacgctccctggcagagtgcagccctgccgtgcagcagccggtatgacctcttccttgtgatcaggagggccctgctgaactgtttccgccccgcaggtgcctacgaagcccgggaaatgatgtggccttcctggagccatgcaatggctttgttgtcaccaggaaaagggcctgtggcacccgcctggccactcatgtcctaaatgagacaggccctcttcatcggcctcagtggctcattgagatgaggacttgggaattttgctgtttaacagagcaactgagcacccaggtggctgccccagcagaccctggagacgtttcaggagacctggcagggacccaagcctctgccactgcaccaggccctggccagagggctgggctcagagccctttatttttttatttttattttttattttttagagacacagtattgccctgtctcccaggctggagcacagcagttgaaaccatacctcactgcagcctcgatctcccaggcttaaatgattctcctgcctcagcctccaagtagctgggaccacaggcatatgccaccatgccagccttattgttaaatgttttgggtagatcccatctccctatgttgctcaggctggtcttgaactcctgggctcaagcgttcctcacatctcagcctcttgagtagctgagaccacaagtgtgtgccaccgcacctggccccagagccccttttaaactgcaactcacagtctccaagttagactcacacagagaagatctaaatatgtgtctccttgagggaggctgaggagtggaggaggatgaactcttacaaaacatcaacctttttaaaaatgtgttttcagtaattgctgttctgcgccaagttttatcctagtgggagtttcatgtcagaattactaagtaggagttcataacagagaagttaatcgcccttgtgtaggggcgaggcaccgagcgatgatctctgtgcccaggtaggtgcttcctggatccgcacaagcacaggagatggcaggtggggagtgggtggggggttatgaagggcagccgaggaggggcagggggcagggggaagcaggatctctgacggtagaagggagtggtcactacgtccccaacacacccccttcatgtccccgctatagccacacaccacgggggaaaggctccaggccagcccccatcccctcaggaccatgatgcgggcatctgcagaaacgggtgggggctgtctggcctgagaggcctagagccaggaacaggtggtttagagctgccctcctcctccaacttcagccccaacccccttcctcagcagcagatcccacctgagtctctcctaggcctgttctggatccgaagtgggtatgagacattcaccatctattcctttgctccaccgtcaccagaggctttgtggtaccttatttttgagaagaggcaacatattctaggactaggctgggaacaagggagaagttcatcatgcatccctccatttatccatccatccatccatccatccatccatcatccattctcccacctacccac

SEQ ID NO: 13862 - RNA, 5609 nt, Homo sapiens
  source 1..5609: mol_type = other RNA
gctgggattacaggcatgagccaccatgcctggctgtaattcaatttttaaagggaaatttaaaaatagtataaggctcaaaggttcaattaaagaaaccatttatgaaggagaataataaaatattactttgtgtacatatgtcagtgcagagaattgggtaagggtgatttttagctctgttaagacttgcttcagaatgccataccacagtctgaaagaatcatatgaaagtaagatattattttaaaaacaaaagtgccgggcacggtggcttaagcctgtaatcccagcactttgggaggccaaggtgggtggatcacctgaggtcaggagtttaagaccagcctggccaacatggtgaaaccctgtctccattaaaaatttaaaaaattagctgggcgtggtggcgggcaccggtaatcctagctattagggaggctgagacatgagaattgcttgaacccaggaatcagaggttgcagtgagctgagattgcgccacacactccagcctgggcgagagagcaagactccgtctccaaaaaaaaaaaaaaaaaaaaaaaaagggtcacaattccctaaagcctaaaactggataaaatgtgcactaacaaaaatgaatatttagaagtattcaactagttttgttcactatgaaaaataattttaagttgtagaagcattatttcattcaacattttgttacatcacaaaatttttaaatgactaaattttaaacaatatttaaacaaaaatatttacttcacattttaattcaatgcaaattttcactaatttagaagtctatgttaatacagattgagtataccctttccaaaatgcttgggaccagagtttctcaggtttcagactttttcagattttggaatatgtgcagaaatacagtggttgagttttcctaatccaaaaatctgaaatgcaaaatgctccaatgaacatttcctttaaagtgtcacatcggcactcaaaaatgttcttatctgaagcattctgaattttggattggggtgctcaatggctgtatgagtatttggggaattcctggaaatggacacattattacatataaaactgtcttacagaccttagaaataaggttttacaatggttcataagctttacaaatcttcctaaactactttttaaaaaacaatgcttaattatatagattttgattttttttttttttttttttgagacggagtctcactctgtcacctaggctggagtgcagtggcacgatcttggctcactgcaacctctgcctcccgggttcaagcgattctcctgcctcagcctcccaagtagctgggactacaggcgcccgccaccatgcccggctaatttattgtatttttagtagagacggggtttcaccatggtcttgatctcctgatctcgtgatccacccgcctcggcctcccaaagtgctgggattacaggcgtgagccaccgcgcccggcccagttctgtttttttgttttgttttgttttgtattttgtgtttttcttgagatggagtttcactcctgttgcccaggctggagtgcaatggcgcgatctcagctcaccgcaacctctgcctcctgggttcaagcaattctcctgtctcagcttccccagtagctgagattacaggtatgcaccaccatgcctggctaattttgtattcttagtagagatggggtttctccacattggtcaggctggtctcaaactcccaacctcaggtgatccacctgcctcggcctcccaaactgctgggattacaggcgtaagccaccatgcccagcctgttttaaaaattctaatgaactggcctggtgcggtggctgacacctgtaatcccggcactttgggaggctgaggcgggcggatcacgaggtcaggagatcgagaccatcctggttaacacggtgaaaccccatctctactaaaaatacaaaaaattagccaggcatggtggtgggcgcctgtagtcccagctactcgtgaggctgaggcagaagaatggtgcaaacccgggaggcagagcttgcagtgagccgagatcgtgccattgcactccagcttgggtgacagagtgactctgtctcaaacaacaacaacaaaattctaattaataattagattggaaatcattatttaaaaaattagttatgactcagaaaatattattatataaaaattcaaggagaggacattattagggtcatcttaccattattagccatagcagtactgtgtcttgcacacatctacaaatcatggttttttttttttttttttttttttttgagagagtcttgctctgttacccaggctggagtgcaatggcacaatcttggctcactgcaacctccacctccaagggttcaagcgattctccctgcctcagcctcctgagtagctgggattatacaggcgcctgccaccacgcccggctaatttttgtatttttagtagagacggggtttcgccatgttggccaggctggtctcaaactcctgactcaagctgctcatccactttggcctcccaaagtgctgggattacaggcgtgagccactgtgcctggcctacaaatcctgtttttaaactgacaatctgttctaactactttgctcattagcacacgaaaatgatactggttgagttcgaaacattgtaatttgtatttatagaaaccctaagtaagatagttcccaagattaaatgctattttaaaatactttttggaacaaaaatacctcattttatcttatatcattaggagtaaacatgatccatataagtgatttttaaaattcataccttaaagcaatgatagtttttaaaaattaaaccattttttaatagaggtgatcttaaaataccttcatttattgccttgtaaaattctacctcctggtcctgacccccaagctttctgtgaaagattccagggtcaacactatgaatgtcaaatattataatccattataacaaagtattaacctcagcaatttcttaagtgtaacaaatgtttatcttacggttgctgcttctgtaggcatagatatttcctgattacttcatattattctaacttctagaagtcctgtccctctggtgcttctcacctgtttttaaaaaaatcagtacatgtaattttctacattattctagctcaaaagtgctccacactttttctgcagcttaaaataagtttttctttctttccttttgggattaggggaaaggaagacggctgggcttgataacacactcatttgtaggtttgcttcagaggtgctggatatttcctgatgggtaagtttgctaaagaaatacataccaagaggtcgccatgttatcatactgaggacagcaggaaactcttccaggtgagaccagaaaggataatacaataatttgctaatagttaacagacatttgatattttatggacataaataaaatgatttacctactttacaaagtaatattaactacaggtgtatctaaaaacctatgaaattatttgcaacaaatatttcactgataaaaatttcttaatatttcccttagcaaaaactgtacatttgttagagagtacctgatacttgttaaaatatcaagtaatacaggacatggtgctgtaaaacaaaacacacaactgggaagtattttattttttctacttcatataacattgttcaacaccacaagattttaaaggtctctttccccaacttttatgatttagaagtaccacttaaaaatatttactgatgctgtaaatattactgtttttgtacatagtaaagattttaatgaatgccatatccattatacctcttgctcctttggtcagaaagataaacagaaactttaaatcagatgtttggacattcaaaaatggttttgaaaagtatacccaaacaaaccaaatatatatcagcaactattaaaaatcagttttagtagttattaagaattcttaacaaggaagtatcgaagcatgtgtgagattttaaaaactatatacaattttaaaaacaaatttaaatttttaaataaaaaagattaatggccaaattaaaaagtttgtgcatcagatttaatatcttaatgtttatcagaaatatattttgtgagtaagaattatttcataaatatatatgtataaatataaatatatatctgcaggatctgtgatgctggagaaaacattttgaagaaaaaaattgcacttttgattatcaagatattgtcaaatttaccctttaagtgaaatataattaccaatccaggtgcttttggcacaagtttttaggtgaatatcgacacaatcttaaaaacacaatgcttttgtattttattcactggaatatggagaatcaaacagaatttaaaattctgacccaaaaatcccagataactgcaattgcttaattaaatacaaaaaaaaattgttttaaaaagcgcttagacttccctttccatctggaacatgtaaaattttgcagcaacaggttttctccaattccttcagcaagaattcccagcctacacacaaatttaacaccatctttttctattcatgtataacttggatcacacaccagtatataacgacaaaaaataaatgtataataaaaagattggataaatcagaagaggctttttggtcttgaattcttcacccactaacaatgaagcagcactgtaggcagcccaaaacacaccaaacagttttataagtgtagacaccacttcaaatgatccaaccaccaaaagtacaggggctattacaatgagaggaagtaatgaatatcctataactccaaggacttggccatatgcaacttctccaccaagaactctggccagtaagaaaattgttagtgaaccaaatatccaaatggttataatccatgagaccaccctaaactgtccatataatgatatcatggaaaagaaaagaacaacagccagaggaccccaaaagtcaggattgtctctcaccacttgtctattaaaaccaagtgatggcattggcatcaaaacacatcggattttgtagtaaatatcctttagatcaatgtccaattcttccaagagtggcttgttatcttcaggatcatcatcttcaacttccagaagccagccataacctctttgtctcagaaatgtagtagctgtagattctttgataaaatctccaccaagatttaatttgacatctggggatgctattgaaccactgagatcttccgcgtctgctgaggagacaaaggtgaagtccccgttagtgggggcataggccgggggcgggcccggaggctgcatctcgcggcgactcccaaccggccgcggtagaagaggctgcggctgggcccagaccccgaggcggccgcggcggcgacccgcacgctcgccctacggtgcggcctacgagtctcgacgtgcaagctgcgagcgaggccagaaacgggcacagcgggccgctgagctgccccgagactaccccaccaaagtcttcttggtggcgaccacccaagcaccacgacgccggcaccctgacaggaccataacagtgac

SEQ ID NO: 13863 - RNA, 4499 nt, Homo sapiens
  source 1..4499: mol_type = other RNA
gctgggattacaggcatgagccaccatgccttgccaacagcatgtctctatggcacttagggtgcataaatagccaggagcatcccagcatctttttcatgctgagttaagactattaaatccacctcctggaagtccatgcagtgcccatcttcaaaagaggtcagagattgtccacaagccaagtagccaaatgaccaatttattaaagccattagccactgatgggctggggctttcttagtgggctggggctgacatttctgtatcatagtctgttgtcttttatacattcaaaaattaatttccatcgttcagacaggagtacgaagagcagattgataaagtggaaaggaagcacattccagaatcagacctcggagcagttcctcaatctctctgggcctcagtttgcctatttgtaaagatggaaatctccctcatgaggttgttgtaaaggcaacattacataatggcaccaataccattagataacattagataaaacacaaagcctggcacatggtatgtgctcagcatgttttaaaaatgcataggagtgccctctgtataccagacactatacaagcactagagacactgtatacaataatgcatagaccttgttccttagacgctggtaatttatatttattgaccatttcttgttcttgtcagactcaaatccaggtctctctgacccagaggcagagctcacaatcagttctctccactagttgccttgattgttcaaggtaaataatggacacttagccacttgtctgtgtgaagtgctcttttcgagtgttctttggtcctgagggaccctgaggagcaactctctcacagggaggtcttctgaacaatggtttctgacctggaaacagaccagctgcagcttctgaaaccgggattaaagtctcctaaactccccccgttttgaacaagaagtttgggggatgcaaagcagagtgagaatgaagctttttacaaaaagtaaatccttttgaaaagacatttacaaatgtgatgagaaaccaaagagaaagcccatatcaaactctgttaacatttgatggtacatttcaaaacatcttcttagtccaagagactcagaaaggtagaaataaataaatcacatagagtatgcttttaaacatcatattttaggcaggtaaaaatatctcactttgacagatcatgcaaagaggaacacaaaatacaaaacatcagcttgtacaggcactccatatgctatacatattgtggtttagcaccaagctttaaaatataaatcacaaccagattgcaacataaacaccaagtaaaactacatgttcctatgtctttactagtttttgcttaccaggtatggctatgaaagattacaatgactttttgacaaacacaacagaactcacagataaaaatgcacttggttccttcaaagcgtccccttccgtaggtgcacgggaactccatgtcagctgttcgtctactcaaacatatcattttgagctgccaccactcttgggaataccgtgtatgtgtatctgtgcacacttaagagggcacattgttaaaatattgtatttttttttttgagacagagtcttgctctgttgcccaggctggagtgcagtggcgtgatcttggctcacggcaacctccacctcccgggttcaagcaattctcgtgcctcggcctcccaagtaagtgggactacaggcatgccccaccatgcccagataatttttgtgtttttagtagagacaaggtttctccatattggccagactggtcttgaactcctggcctcaaatgatctgcccacctcagcctctcaacatgctgggattataggcttgagctaccatgcccggccaaaagggcacatttttgcctttcggagaaaatatgctacaataagctgaaaccccagaggatctgtactctaactttctcacataactagctatgtgaccttgggtacctctctcaccttgctgaacctcaatttgctcctctgcaaactagagttagaaaattaccctcctgtggggtgttgtggggcttaaatgagataaacctagtacagccctcaaaaatatggcattctgcccccattccttcttttaatttttaacgtgcaaccattcaaaaatatttcatttctctttcttttgaggatgtcttttgccaccacttttttaatagccaaaggaaatttggggttaaagacgatgggtgtgcaagctgcataattttctatccactctaaacatgtttgagtaagaaataataaggcagaatttccagggtggttcagacactggttctggagaaagctgttaaagaggctcagaagagaagttttctgagaagggatagcccctgtggaacagctgtcatgcctctcaaggtgacccctggaaggggacagcaactattggcatggataaagtctctgcacagttatacagctccattccaggagggctcaagagtccttttcaattctccagtggaaccctagccacgtgtctcttcagttgtcaatcacttgactcggaaagcttgaattacaatgagtctgaggctcccatagttcctgaggagcaggagagttccacccaggtctgattctctctctcttttatttttattatttttttctttttgaacccagttacaagaaacaggtctgactttcttgcaaagattctgcttcctcctcaaagttcaatctctctgctgatcaccgccatctgctgttcttctatggtgcctaagaactttccaaactaccaagcccctaagactgtggtttggattccagaaagcccaggtgcctgcctggcaacacacaggccttcgtcctctatttccttgttggacatcataaggatcattttgttgcatcccctcagagcctcccttaggagcgaatatgcagaattctcttgaatgtcttcttgaagttctcattgcacaaggggtagatgagggggttcagtgtggagttgatgtagcccagccagatggtgaacatgtgcaaatgttcattgcaacagttcttgcagaaggcaatgaccatgaagaagatgaaataagggatccagcagaggatgaaggctgccatgataaaacccaactgtttggcggccttcctttcgcggttcatgtgcaacccagatacatactgtcttgaatgcgagcggagcctcttccaagtaaacttgatgtaatccaggcctgtgttagacccactcctcaatttgcctttgcctggtgctgtctctgtggtggtatctgagtccgttcgagagaaggattggctatcacctaacatctgatcctctgatatctcgctggccccatgtgtgttcaggccctgctcatctgtcttgagctggccatggctccggttgacggctacatagtccctgctactcccctctgccgcagcctgcatgtgcacaatatcaagtggaaagcagtagagtttgtctacttctctatcatcctcttggctgaagacaactggggatttcatctccttgggggtttgggatggtgacttcaagacagatccaccaccagcatcttttggcttccttttcagaacctcccagggagactccttccctggtttcttggcatcccccttggggttctctggcctcagcttaatttctgagaaggaagggagggacctattgatgagctcccggtgctggcagtgttgtcgtacggccttgtagatcttggcatagaaccagagcatgagcaaggtgggcaggtagaagttgatgatggcagtcatgaccttgaaccaggtgacatcatagaagtctgtctcacacttgtcctctcggcgcaccgaggtctgctgcatgaagtgattccagcctagaatgggaataacccacagaaaagagagaaaccaggcccccagaatggtggccgaggctcgggtcttggtacgatacttaaggtacctgaggggctgctggacagagcggtagcgatcaatgcacaggatgaagacactgaaaatggacgctgtgctggccacatagtccatggaaagccaaaagaggcagagaggacggcccagtgaccacttggacatgagcaggtagaggatgttcataggcatgacgacggcacccacgatcaagtccgccaccgagaggctgacgatgtacaggttccccacagtgtggagcttccgctcactccgtacggcatacagcaccagcaggttgagccctactgtgaccaagcagatagtgctcaggaccaccaccaggggcatcagctgggggctggccatagtggtcttgttgccctcacacatcttgtcttctaagaggcaggaggaattggggaggctcattggcgcaagagcagccaccagttatggctcactcccggcgccggctccggggaaagtttggtggcgcgttggccgcggcggccaggctgctgggtgt

SEQ ID NO: 13864 - RNA, 4599 nt, Homo sapiens
  source 1..4599: mol_type = other RNA
gctgggattacaggcatgagccaccatgccttgccaacagcatgtctctatggcacttagggtgcataaatagccaggagcatcccagcatctttttcatgctgagttaagactattaaatccacctcctggaagtccatgcagtgcccatcttcaaaagaggtcagagattgtccacaagccaagtagccaaatgaccaatttattaaagccattagccactgatgggctggggctttcttagtgggctggggctgacatttctgtatcatagtctgttgtcttttatacattcaaaaattaatttccatcgttcagacaggagtacgaagagcagattgataaagtggaaaggaagcacattccagaatcagacctcggagcagttcctcaatctctctgggcctcagtttgcctatttgtaaagatggaaatctccctcatgaggttgttgtaaaggcaacattacataatggcaccaataccattagataacattagataaaacacaaagcctggcacatggtatgtgctcagcatgttttaaaaatgcataggagtgccctctgtataccagacactatacaagcactagagacactgtatacaataatgcatagaccttgttccttagacgctggtaatttatatttattgaccatttcttgttcttgtcagactcaaatccaggtctctctgacccagaggcagagctcacaatcagttctctccactagttgccttgattgttcaaggtaaataatggacacttagccacttgtctgtgtgaagtgctcttttcgagtgttctttggtcctgagggaccctgaggagcaactctctcacagggaggtcttctgaacaatggtttctgacctggaaacagaccagctgcagcttctgaaaccgggattaaagtctcctaaactccccccgttttgaacaagaagtttgggggatgcaaagcagagtgagaatgaagctttttacaaaaagtaaatccttttgaaaagacatttacaaatgtgatgagaaaccaaagagaaagcccatatcaaactctgttaacatttgatggtacatttcaaaacatcttcttagtccaagagactcagaaaggtagaaataaataaatcacatagagtatgcttttaaacatcatattttaggcaggtaaaaatatctcactttgacagatcatgcaaagaggaacacaaaatacaaaacatcagcttgtacaggcactccatatgctatacatattgtggtttagcaccaagctttaaaatataaatcacaaccagattgcaacataaacaccaagtaaaactacatgttcctatgtctttactagtttttgcttaccaggtatggctatgaaagattacaatgactttttgacaaacacaacagaactcacagataaaaatgcacttggttccttcaaagcgtccccttccgtaggtgcacgggaactccatgtcagctgttcgtctactcaaacatatcattttgagctgccaccactcttgggaataccgtgtatgtgtatctgtgcacacttaagagggcacattgttaaaatattgtatttttttttttgagacagagtcttgctctgttgcccaggctggagtgcagtggcgtgatcttggctcacggcaacctccacctcccgggttcaagcaattctcgtgcctcggcctcccaagtaagtgggactacaggcatgccccaccatgcccagataatttttgtgtttttagtagagacaaggtttctccatattggccagactggtcttgaactcctggcctcaaatgatctgcccacctcagcctctcaacatgctgggattataggcttgagctaccatgcccggccaaaagggcacatttttgcctttcggagaaaatatgctacaataagctgaaaccccagaggatctgtactctaactttctcacataactagctatgtgaccttgggtacctctctcaccttgctgaacctcaatttgctcctctgcaaactagagttagaaaattaccctcctgtggggtgttgtggggcttaaatgagataaacctagtacagccctcaaaaatatggcattctgcccccattccttcttttaatttttaacgtgcaaccattcaaaaatatttcatttctctttcttttgaggatgtcttttgccaccacttttttaatagccaaaggaaatttggggttaaagacgatgggtgtgcaagctgcataattttctatccactctaaacatgtttgagtaagaaataataaggcagaatttccagggtggttcagacactggttctggagaaagctgttaaagaggctcagaagagaagttttctgagaagggatagcccctgtggaacagctgtcatgcctctcaaggtgacccctggaaggggacagcaactattggcatggataaagtctctgcacagttatacagctccattccaggagggctcaagagtccttttcaattctccagtggaaccctagccacgtgtctcttcagttgtcaatcacttgactcggaaagcttgaattacaatgagtctgaggctcccatagttcctgaggagcaggagagttccacccaggtctgattctctctctcttttatttttattatttttttctttttgaacccagttacaagaaacaggtctgactttcttgcaaagattctgcttcctcctcaaagttcaatctctctgctgatcaccgccatctgctgttcttctatggtgcctaagaactttccaaactaccaagcccctaagactgtggtttggattccagaaagcccaggtgcctgcctggcaacacacaggccttcgtcctctatttccttgttggacatcataaggatcattttgttgcatcccctcagagcctcccttaggagcgaatatgcagaattctcttgaatgtcttcttgaagttctcattgcacaaggggtagatgagggggttcagtgtggagttgatgtagcccagccagatggtgaacatgtgcaaatgttcattgcaacagttcttgcagaaggcaatgaccatgaagaagatgaaataagggatccagcagaggatgaaggctgccatgataaaacccaactgtttggcggccttcctttcgcggttcatgtgcaacccagatacatactgtcttgaatgcgagcggagcctcttccaagtaaacttgatgtaatccaggcctgtgttagacccactcctcaatttgcctttgcctggtgctgtctctgtggtggtatctgagtccgttcgagagaaggattggctatcacctaacatctgatcctctgatatctcgctggccccatgtgtgttcaggccctgctcatctgtcttgagctggccatggctccggttgacggctacatagtccctgctactcccctctgccgcagcctgcatgtgcacaatatcaagtggaaagcagtagagtttgtctacttctctatcatcctcttggctgaagacaactggggatttcatctccttgggggtttgggatggtgacttcaagacagatccaccaccagcatcttttggcttccttttcagaacctcccagggagactccttccctggtttcttggcatcccccttggggttctctggcctcagcttaatttctgagaaggaagggagggacctattgatgagctcccggtgctggcagtgttgtcgtacggccttgtagatcttggcatagaaccagagcatgagcaaggtgggcaggtagaagttgatgatggcagtcatgaccttgaaccaggtgacatcatagaagtctgtctcacacttgtcctctcggcgcaccgaggtctgctgcatgaagtgattccagcctagaatgggaataacccacagaaaagagagaaaccaggcccccagaatggtggccgaggctcgggtcttggtacgatacttaaggtacctgaggggctgctggacagagcggtagcgatcaatgcacaggatgaagacactgaaaatggacgctgtgctggccacatagtccatggaaagccaaaagaggcagagaggacggcccagtgaccacttggacatgagcaggtagaggatgttcataggcatgacgacggcacccacgatcaagtccgccaccgagaggctgacgatgtacaggttccccacagtgtggagcttccgctcactccgtacggcatacagcaccagcaggttgagccctactgtgaccaagcagatagtgctcaggaccaccaccaggggcatcagctgggggctggccatagtggtcttgttgccctcacacatcttgtcttctaagaggcaggaggaattggggaggctcattggcgcaagagcagccaccagttatggctcactccctggctggtttcagtagcttcctgtctccagacctcagggcttgcttcttgtagttcatttctccatcagtgcacgagcagagtgatttttcttaaatgaaaaatcccattgagggctgcctggcggacaacttctctacggctactatcaaaagaaaatgc

SEQ ID NO: 13865 - RNA, 4516 nt, Homo sapiens
  source 1..4516: mol_type = other RNA
gctgggattacaggcatgagccaccatgccttgccaacagcatgtctctatggcacttagggtgcataaatagccaggagcatcccagcatctttttcatgctgagttaagactattaaatccacctcctggaagtccatgcagtgcccatcttcaaaagaggtcagagattgtccacaagccaagtagccaaatgaccaatttattaaagccattagccactgatgggctggggctttcttagtgggctggggctgacatttctgtatcatagtctgttgtcttttatacattcaaaaattaatttccatcgttcagacaggagtacgaagagcagattgataaagtggaaaggaagcacattccagaatcagacctcggagcagttcctcaatctctctgggcctcagtttgcctatttgtaaagatggaaatctccctcatgaggttgttgtaaaggcaacattacataatggcaccaataccattagataacattagataaaacacaaagcctggcacatggtatgtgctcagcatgttttaaaaatgcataggagtgccctctgtataccagacactatacaagcactagagacactgtatacaataatgcatagaccttgttccttagacgctggtaatttatatttattgaccatttcttgttcttgtcagactcaaatccaggtctctctgacccagaggcagagctcacaatcagttctctccactagttgccttgattgttcaaggtaaataatggacacttagccacttgtctgtgtgaagtgctcttttcgagtgttctttggtcctgagggaccctgaggagcaactctctcacagggaggtcttctgaacaatggtttctgacctggaaacagaccagctgcagcttctgaaaccgggattaaagtctcctaaactccccccgttttgaacaagaagtttgggggatgcaaagcagagtgagaatgaagctttttacaaaaagtaaatccttttgaaaagacatttacaaatgtgatgagaaaccaaagagaaagcccatatcaaactctgttaacatttgatggtacatttcaaaacatcttcttagtccaagagactcagaaaggtagaaataaataaatcacatagagtatgcttttaaacatcatattttaggcaggtaaaaatatctcactttgacagatcatgcaaagaggaacacaaaatacaaaacatcagcttgtacaggcactccatatgctatacatattgtggtttagcaccaagctttaaaatataaatcacaaccagattgcaacataaacaccaagtaaaactacatgttcctatgtctttactagtttttgcttaccaggtatggctatgaaagattacaatgactttttgacaaacacaacagaactcacagataaaaatgcacttggttccttcaaagcgtccccttccgtaggtgcacgggaactccatgtcagctgttcgtctactcaaacatatcattttgagctgccaccactcttgggaataccgtgtatgtgtatctgtgcacacttaagagggcacattgttaaaatattgtatttttttttttgagacagagtcttgctctgttgcccaggctggagtgcagtggcgtgatcttggctcacggcaacctccacctcccgggttcaagcaattctcgtgcctcggcctcccaagtaagtgggactacaggcatgccccaccatgcccagataatttttgtgtttttagtagagacaaggtttctccatattggccagactggtcttgaactcctggcctcaaatgatctgcccacctcagcctctcaacatgctgggattataggcttgagctaccatgcccggccaaaagggcacatttttgcctttcggagaaaatatgctacaataagctgaaaccccagaggatctgtactctaactttctcacataactagctatgtgaccttgggtacctctctcaccttgctgaacctcaatttgctcctctgcaaactagagttagaaaattaccctcctgtggggtgttgtggggcttaaatgagataaacctagtacagccctcaaaaatatggcattctgcccccattccttcttttaatttttaacgtgcaaccattcaaaaatatttcatttctctttcttttgaggatgtcttttgccaccacttttttaatagccaaaggaaatttggggttaaagacgatgggtgtgcaagctgcataattttctatccactctaaacatgtttgagtaagaaataataaggcagaatttccagggtggttcagacactggttctggagaaagctgttaaagaggctcagaagagaagttttctgagaagggatagcccctgtggaacagctgtcatgcctctcaaggtgacccctggaaggggacagcaactattggcatggataaagtctctgcacagttatacagctccattccaggagggctcaagagtccttttcaattctccagtggaaccctagccacgtgtctcttcagttgtcaatcacttgactcggaaagcttgaattacaatgagtctgaggctcccatagttcctgaggagcaggagagttccacccaggtctgattctctctctcttttatttttattatttttttctttttgaacccagttacaagaaacaggtctgactttcttgcaaagattctgcttcctcctcaaagttcaatctctctgctgatcaccgccatctgctgttcttctatggtgcctaagaactttccaaactaccaagcccctaagactgtggtttggattccagaaagcccaggtgcctgcctggcaacacacaggccttcgtcctctatttccttgttggacatcataaggatcattttgttgcatcccctcagagcctcccttaggagcgaatatgcagaattctcttgaatgtcttcttgaagttctcattgcacaaggggtagatgagggggttcagtgtggagttgatgtagcccagccagatggtgaacatgtgcaaatgttcattgcaacagttcttgcagaaggcaatgaccatgaagaagatgaaataagggatccagcagaggatgaaggctgccatgataaaacccaactgtttggcggccttcctttcgcggttcatgtgcaacccagatacatactgtcttgaatgcgagcggagcctcttccaagtaaacttgatgtaatccaggcctgtgttagacccactcctcaatttgcctttgcctggtgctgtctctgtggtggtatctgagtccgttcgagagaaggattggctatcacctaacatctgatcctctgatatctcgctggccccatgtgtgttcaggccctgctcatctgtcttgagctggccatggctccggttgacggctacatagtccctgctactcccctctgccgcagcctgcatgtgcacaatatcaagtggaaagcagtagagtttgtctacttctctatcatcctcttggctgaagacaactggggatttcatctccttgggggtttgggatggtgacttcaagacagatccaccaccagcatcttttggcttccttttcagaacctcccagggagactccttccctggtttcttggcatcccccttggggttctctggcctcagcttaatttctgagaaggaagggagggacctattgatgagctcccggtgctggcagtgttgtcgtacggccttgtagatcttggcatagaaccagagcatgagcaaggtgggcaggtagaagttgatgatggcagtcatgaccttgaaccaggtgacatcatagaagtctgtctcacacttgtcctctcggcgcaccgaggtctgctgcatgaagtgattccagcctagaatgggaataacccacagaaaagagagaaaccaggcccccagaatggtggccgaggctcgggtcttggtacgatacttaaggtacctgaggggctgctggacagagcggtagcgatcaatgcacaggatgaagacactgaaaatggacgctgtgctggccacatagtccatggaaagccaaaagaggcagagaggacggcccagtgaccacttggacatgagcaggtagaggatgttcataggcatgacgacggcacccacgatcaagtccgccaccgagaggctgacgatgtacaggttccccacagtgtggagcttccgctcactccgtacggcatacagcaccagcaggttgagccctactgtgaccaagcagatagtgctcaggaccaccaccaggggcatcagctgggggctggccatagtggtcttgttgccctcacacatcttgtcttctaagaggcaggaggaattggggaggctcattggcgcaagagcagccaccagttatggctcactccctttacaaatgctgctctcctgccgggaatgcctgttctcatcctcttaccctggcaagacattcagttagttctttac

SEQ ID NO: 13866 - RNA, 1178 nt, Homo sapiens
  source 1..1178: mol_type = other RNA
gctgggattacaggcatgagccaccatgccttgccaatgattctaatttatatttttaaaaattaccctataatcttaaaacttttaactgactagtatccaacccttaaacttcataacaatcatttccaaagtggaaaagtcactgggatatggggacagtatgatttgtctttatacttttatttttctaacatctttttgttttctagtatacatgttagcacaggagtatgtatattacttaagtatgcctatgttggggtgcagacataatttctttttaaatgataggatgcaaaatcaaatctgtttgcataccagtgaagaggctatttctcaatcttggcaaactagggggtgcatacccccttcttttattcagtagcttccataaggatgtaacttacggaagttatatccttccataaactgataggctatccaaccagtgaggaaaactgataaagtggcttctgagctccaagtagcagttaaacacaactaaatatatcttgaaagtttggaaaaaaatttaacagtaaagggattcagtagttattcagtataaggtttggaattcaaaaactccagccattacaatagacatttatttaaagtaaaacatcttcagaccaaataattcttaaaattgtttgtttcaagtttaaccatcttcataacagctgcatccacagacttcaactacatgattacttctttgcccattcttctctttcttttctttcccgaataacctctttcagatacggttcaaggtagaaattttcctcttcatatttggtccactgctctttaggcaagatctgatgcttcaagttcaggtccagtgccctcttaatgcgaaacatcctgtcattataaaggttctcaggaagtcttcttatggcttcttttacatcttcatcctcgtatattgtatcatctcgcattaaccccagtttattgaatcctgcagcattgtaataccattttcgaataccatccagccacttgcctgatgctgaaaagaagtgatcccacccaaggtcagagttagctaatgggagttgagatctggtctatgtagttcccaaacacgcacagaagcagtgtcttgaatttagtaagactccttcaatatcggcctgcttaccagccattttgaccagaaagag

SEQ ID NO: 13867 - RNA, 1064 nt, Homo sapiens
  source 1..1064: mol_type = other RNA
gctgggattacaggcatgagccaccatgccttgccaatgattctaatttatatttttaaaaattaccctataatcttaaaacttttaactgactagtatccaacccttaaacttcataacaatcatttccaaagtggaaaagtcactgggatatggggacagtatgatttgtctttatacttttatttttctaacatctttttgttttctagtatacatgttagcacaggagtatgtatattacttaagtatgcctatgttggggtgcagacataatttctttttaaatgataggatgcaaaatcaaatctgtttgcataccagtgaagaggctatttctcaatcttggcaaactagggggtgcatacccccttcttttattcagtagcttccataaggatgtaacttacggaagttatatccttccataaactgataggctatccaaccagtgaggaaaactgataaagtggcttctgagctccaagtagcagttaaacacaactaaatatatcttgaaagtttggaaaaaaatttaacagtaaagggattcagtagttattcagtataaggtttggaattcaaaaactccagccattacaatagacatttatttaaagtaaaacatcttcagaccaaataattcttaaaattgtttgtttcaagtttaaccatcttcataacagctgcatccacagacttcaactacatgattacttctttgcccattcttctctttcttttctttcccgaataacctctttcagatacggttcaaggtagaaattttcctcttcatatttggtccactgctctttaggcaagatctgatgcttcaagttcaggtccagtgccctcttaatgcgaaacatcctgtcattataaaggttctcaggaagtcttcttatggcttcttttacatcttcatcctcgtatattgtatcatctcgcattaaccccagtttattgaatcctgcagcattgtaataccattttcgaataccatccagccacttgcctgatgctgaaacggcctgcttaccagccattttgaccagaaagag

SEQ ID NO: 13868 - RNA, 1201 nt, Homo sapiens
  source 1..1201: mol_type = other RNA
gctgggattacaggcatgagccaccatgccttgccaatgattctaatttatatttttaaaaattaccctataatcttaaaacttttaactgactagtatccaacccttaaacttcataacaatcatttccaaagtggaaaagtcactgggatatggggacagtatgatttgtctttatacttttatttttctaacatctttttgttttctagtatacatgttagcacaggagtatgtatattacttaagtatgcctatgttggggtgcagacataatttctttttaaatgataggatgcaaaatcaaatctgtttgcataccagtgaagaggctatttctcaatcttggcaaactagggggtgcatacccccttcttttattcagtagcttccataaggatgtaacttacggaagttatatccttccataaactgataggctatccaaccagtgaggaaaactgataaagtggcttctgagctccaagtagcagttaaacacaactaaatatatcttgaaagtttggaaaaaaatttaacagtaaagggattcagtagttattcagtataaggtttggaattcaaaaactccagccattacaatagacatttatttaaagtaaaacatcttcagaccaaataattcttaaaattgtttgtttcaagtttaaccatcttcataacagctgcatccacagacttcaactacatgattacttctttgcccattcttctctttcttttctttcccgaataacctctttcagatacggttcaaggtagaaattttcctttgcctagtttcaatgcagttcaaggggtgagagtttgcttcacagaagctcttcttgggatctggagggacactcaatgggctgatcttttcatctaagtaggaagcagagtgcagagctggaacagcaaagacctcttcatatttggtccactgctctttaggcaagatctgatgcttcaagttcaggtccagtgccctcttaatgcgaaacatcctgtcattataaaggttctcaggaagtcttcttatggcttcttttacatcttcatcctcgtatattgtatcatctcgcattaaccccagtttattgaatcctgcagcattgtaataccattttcgaataccatccagccacttgcctgatgctgaaacggcctgcttaccagccattttgaccagaaagag

SEQ ID NO: 13869 - RNA, 1354 nt, Homo sapiens
  source 1..1354: mol_type = other RNA
gctgggattacaggcatgagccaccatgccttgccaatgattctaatttatatttttaaaaattaccctataatcttaaaacttttaactgactagtatccaacccttaaacttcataacaatcatttccaaagtggaaaagtcactgggatatggggacagtatgatttgtctttatacttttatttttctaacatctttttgttttctagtatacatgttagcacaggagtatgtatattacttaagtatgcctatgttggggtgcagacataatttctttttaaatgataggatgcaaaatcaaatctgtttgcataccagtgaagaggctatttctcaatcttggcaaactagggggtgcatacccccttcttttattcagtagcttccataaggatgtaacttacggaagttatatccttccataaactgataggctatccaaccagtgaggaaaactgataaagtggcttctgagctccaagtagcagttaaacacaactaaatatatcttgaaagtttggaaaaaaatttaacagtaaagggattcagtagttattcagtataaggtttggaattcaaaaactccagccattacaatagacatttatttaaagtaaaacatcttcagaccaaataattcttaaaattgtttgtttcaagtttaaccatcttcataacagctgcatccacagacttcaactacatgattacttctttgcccattcttctctttcttttctttcccgaataacctctttcagatacggttcaaggtagaaattttcttttgaatttccaattttagaaaacatattctcaacctaagaactatctgctttttaaaatgtcaaatctgtggtgatggtgtgataagttgctttgataggttatgagggggaagtcttttcgggaagaaaaagaaatgaatgtccacaggcctttgcctagtttcaatgcagttcaaggggtgagagtttgcttcacagaagctcttcttgggatctggagggacactcaatgggctgatcttttcatctaagtaggaagcagagtgcagagctggaacagcaaagacctcttcatatttggtccactgctctttaggcaagatctgatgcttcaagttcaggtccagtgccctcttaatgcgaaacatcctgtcattataaaggttctcaggaagtcttcttatggcttcttttacatcttcatcctcgtatattgtatcatctcgcattaaccccagtttattgaatcctgcagcattgtaataccattttcgaataccatccagccacttgcctgatgctgaaacggcctgcttaccagccattttgaccagaaagag

SEQ ID NO: 13870 - RNA, 4115 nt, Homo sapiens
  source 1..4115: mol_type = other RNA
gctgggattacaggcatgagccaccatgccttgccttaacttttatatcgtgtgtgatgaatttatatcatggtgtgaattttctggagcattttacaggcagagattgcttaatcatgggtatatgttctgagaaacgtgttgtaggtgatttcctcatggtacaaacatcacaaagtgaacttacacaaatctagatggtatagctacaacacatctagactatatggtacagtctattgctactaggctataaaccatacaacatgttgttgtactgaacactgtaggaaattgtaacaaaatgttaagtatttatgagtctaaacacagaaaatacacagagtaaacatgcagtataaaagataaaaaaggatgcacctgcataggacactccatgaacatagcttgcaggactagaagttgctctgggtgagtcagttgagtggtgagtgaatgcgaaggcccaggatgttactgtacactaatggagaatttataaacactgtacacttggactacactacattcataaaaacattttttcctcaataatgaataaaccttaacttactgtacattattttctttataaacttatttttaaaaactttgtaataatttagcttaaaacacattgtacagctgtacaaaaatattttatgtccatattctataagctttttctattaaatttttttaaactatttttgttaaagactaactaagacacaaacacacattagtgtaggactacacggggtgaggatcatcaatatcattgtcttctgcctccatgttttgtcccgccagaatacgttcaggggcagtcctgcacatggagccgtcatcgcctatcataacaaagtttttccgggaatatctccttaaggacctgcctgagactgtcttactgttaaaaaaacacaggaatacattctaaaacaggattgtaaatatataaaccagtaacttagccatttattatcaagtatatattgcacatctgtgctgtaattttttttttttcgagacggagtctcgctctgtcacccaggctggagtgtagtggtagatctcagctcactgcaatctccacctcccgggttcaagcgattctcctgctttggcctcccaagtagctgggactacaggcacaccagaacgcccagctaattttcgtatttctaatggagacagggtttcatcatgttgaccaggctggtcttgaactcctgacctcaactgattctcccacctcagcctcccaaagtgctgggattacaggtatgagccactgtgcccagccaattttttttttttttttttgatacagtctcactgtcacccatgctggactgccatcacgtgatcttggttcactgtagccttgaactcctgggctcaggcaatcctcctgcctcagcctcccatgtagatgggactacagggtgtgctaccacacttagaaaatgtttttattttttgtagagacagggtctcactaggttgaccagagtagtcctggcatcaagcaatcctactgccttagtctcccagtgttgggatcacaggtgtgaccatgcccagctgtgttgtactttttttttttttttttttttgagacagagtctcgctctgttggccggatctcagctcactgtcagctcggcctcctgggtttatgccattctcctgcctcagcctcccaagtagctgggactacaggcgcccaccaccacgcccggctaattgtttgtatttttagtagagatggggttttaccgtgttagccaggatggtcttgatctcctggcctcgtgatccgcccgccttggcctcccaaagtgctgggattacaggcgtgagccaccgtccccggccgctgtcttgtacttttatacaactgaaagtgcagcacgtttacaccagcaccataaacacttaaataatgtgctgcactatggtgttactactgctactaaattgcggttgatagaaatgttttaggtgttatataatcttatggggctaccaacctatatggtccattgctgactgaaacatgattatgtggtacctgactatacatgaatcatcttgtatctcgctttctatattacttacattgacaggatttctctcttcagtgggaattttcacaactttgaaagcatctgttagaattgaaaactttctcctatttctcacatttatagagtttctatcgattgtgcattctcatatgtttttttaaggatgtggacacactgaaggcttttccacattgcttacattcaagaggtttctcataattgtgaattcttgtatgtctttgaaaggaactgtgaagactaaaggccttcccacattctttacatttatagggtttctctccagtatgcattctcatgtgtccttgaaagcttgtgggataaataaaggccttcccgcattccttacattcataaggtttctccccagtgtgagttcttttatgtatccgaatgtaactagaacaactaaaggcttttccacattgtttacattcatagggtttctctccagtgtgagttctttcatgtgttcgtaacgcactaggaaaaatgaacaccttcccacagtccctacatttataaggtccgtctccagtgtgggtgatcatgtgtcttcgaaagttctcaagagaaatgaaggtttttgcacattccttacactcatagggtttttctccagtgtgatttctcttgtggattttcaaatctagaggataattgaaagttttcccacattttttacattcgtagggtttctctccagtgtgagtcctttcatgtattcgaaagtaactgattctactaaaggctttcccacattctttacacttatagggtttctctccagtatgcactctcacgtgtactcgaaaggctgggcgtgcactgaaagatttcccacattctttacatttatagggcttctctccagtatgaattctttcatgaatttgaatggaggtggaacatctgaaggctttaccacattgtttacatttatagggtttctctccagtgtgaattctttcatgtactcgtaaaaaactgggaaaaatgaatgcctttccacattctttgcatttataaggtctatctccgttgtgtgttatcatgtgtgttagaacacttgtgtgggaaatgaaggctttcccacattccttacatgcatagggtttctctccagtgtgagttctttcgtgtactcgaatagaactggaacaactgaaggctttcccacattgtttacattcatagggcttttctccagtgtgaatcctttcatgaactcgaagcgaactggaacaactaagagcttttccacattgcttacattcatagggtttttctccaatgtgagtccgctcatgtctttgaaagggctggtgatatatgaaggtttttccacattgtttacatttatagggtttttctccagtgtgactcctttcatgtctttgaaaggatttgagataactaaaggctttctcacactccttacatttatatggcttctcaaatagctcgtatccagtgtgagacctcatgtgtctagtaagggatgagagacgcatgaaggcttttccacagatagtacactcatatggttttactccggcagtcttcttcgtcacactgagattgggactgaagttttctgcacattgactaccttctttaccttcacagagtctctctcccgtatggcttcttagatttcgtccttggtttttgtgttgatcttcaacattcgggtcttcccatttttcccctatagatgccaggttcttgaatgtttcctgcatcacatctctgtagagtttcttctgtgaaggagccagcagagcccactcctcctggctgaagctcacagacacatcctcaaaagccactgagtccattttccggcctcgcgggtgtcccggtgttgtccctaaggttcacggagccagcgcagggtacagcgcatccgatgcaggggtacagcaacctgacgcgtcaaggggccaggagaccccaagctaagcacaacccgatcgcacagtgacgtagcacgcattt

SEQ ID NO: 13871 - RNA, 4087 nt, Homo sapiens
  source 1..4087: mol_type = other RNA
gctgggattacaggcatgagccaccatgccttgccttaacttttatatcgtgtgtgatgaatttatatcatggtgtgaattttctggagcattttacaggcagagattgcttaatcatgggtatatgttctgagaaacgtgttgtaggtgatttcctcatggtacaaacatcacaaagtgaacttacacaaatctagatggtatagctacaacacatctagactatatggtacagtctattgctactaggctataaaccatacaacatgttgttgtactgaacactgtaggaaattgtaacaaaatgttaagtatttatgagtctaaacacagaaaatacacagagtaaacatgcagtataaaagataaaaaaggatgcacctgcataggacactccatgaacatagcttgcaggactagaagttgctctgggtgagtcagttgagtggtgagtgaatgcgaaggcccaggatgttactgtacactaatggagaatttataaacactgtacacttggactacactacattcataaaaacattttttcctcaataatgaataaaccttaacttactgtacattattttctttataaacttatttttaaaaactttgtaataatttagcttaaaacacattgtacagctgtacaaaaatattttatgtccatattctataagctttttctattaaatttttttaaactatttttgttaaagactaactaagacacaaacacacattagtgtaggactacacggggtgaggatcatcaatatcattgtcttctgcctccatgttttgtcccgccagaatacgttcaggggcagtcctgcacatggagccgtcatcgcctatcataacaaagtttttccgggaatatctccttaaggacctgcctgagactgtcttactgttaaaaaaacacaggaatacattctaaaacaggattgtaaatatataaaccagtaacttagccatttattatcaagtatatattgcacatctgtgctgtaattttttttttttcgagacggagtctcgctctgtcacccaggctggagtgtagtggtagatctcagctcactgcaatctccacctcccgggttcaagcgattctcctgctttggcctcccaagtagctgggactacaggcacaccagaacgcccagctaattttcgtatttctaatggagacagggtttcatcatgttgaccaggctggtcttgaactcctgacctcaactgattctcccacctcagcctcccaaagtgctgggattacaggtatgagccactgtgcccagccaattttttttttttttttttgatacagtctcactgtcacccatgctggactgccatcacgtgatcttggttcactgtagccttgaactcctgggctcaggcaatcctcctgcctcagcctcccatgtagatgggactacagggtgtgctaccacacttagaaaatgtttttattttttgtagagacagggtctcactaggttgaccagagtagtcctggcatcaagcaatcctactgccttagtctcccagtgttgggatcacaggtgtgaccatgcccagctgtgttgtactttttttttttttttttttttgagacagagtctcgctctgttggccggatctcagctcactgtcagctcggcctcctgggtttatgccattctcctgcctcagcctcccaagtagctgggactacaggcgcccaccaccacgcccggctaattgtttgtatttttagtagagatggggttttaccgtgttagccaggatggtcttgatctcctggcctcgtgatccgcccgccttggcctcccaaagtgctgggattacaggcgtgagccaccgtccccggccgctgtcttgtacttttatacaactgaaagtgcagcacgtttacaccagcaccataaacacttaaataatgtgctgcactatggtgttactactgctactaaattgcggttgatagaaatgttttaggtgttatataatcttatggggctaccaacctatatggtccattgctgactgaaacatgattatgtggtacctgactatacatgaatcatcttgtatctcgctttctatattacttacattgacaggatttctctcttcagtgggaattttcacaactttgaaagcatctgttagaattgaaaactttctcctatttctcacatttatagagtttctatcgattgtgcattctcatatgtttttttaaggatgtggacacactgaaggcttttccacattgcttacattcaagaggtttctcataattgtgaattcttgtatgtctttgaaaggaactgtgaagactaaaggccttcccacattctttacatttatagggtttctctccagtatgcattctcatgtgtccttgaaagcttgtgggataaataaaggccttcccgcattccttacattcataaggtttctccccagtgtgagttcttttatgtatccgaatgtaactagaacaactaaaggcttttccacattgtttacattcatagggtttctctccagtgtgagttctttcatgtgttcgtaacgcactaggaaaaatgaacaccttcccacagtccctacatttataaggtccgtctccagtgtgggtgatcatgtgtcttcgaaagttctcaagagaaatgaaggtttttgcacattccttacactcatagggtttttctccagtgtgatttctcttgtggattttcaaatctagaggataattgaaagttttcccacattttttacattcgtagggtttctctccagtgtgagtcctttcatgtattcgaaagtaactgattctactaaaggctttcccacattctttacacttatagggtttctctccagtatgcactctcacgtgtactcgaaaggctgggcgtgcactgaaagatttcccacattctttacatttatagggcttctctccagtatgaattctttcatgaatttgaatggaggtggaacatctgaaggctttaccacattgtttacatttatagggtttctctccagtgtgaattctttcatgtactcgtaaaaaactgggaaaaatgaatgcctttccacattctttgcatttataaggtctatctccgttgtgtgttatcatgtgtgttagaacacttgtgtgggaaatgaaggctttcccacattccttacatgcatagggtttctctccagtgtgagttctttcgtgtactcgaatagaactggaacaactgaaggctttcccacattgtttacattcatagggcttttctccagtgtgaatcctttcatgaactcgaagcgaactggaacaactaagagcttttccacattgcttacattcatagggtttttctccaatgtgagtccgctcatgtctttgaaagggctggtgatatatgaaggtttttccacattgtttacatttatagggtttttctccagtgtgactcctttcatgtctttgaaaggatttgagataactaaaggctttctcacactccttacatttatatggcttctcaaatagctcgtatccagtgtgagacctcatgtgtctagtaagggatgagagacgcatgaaggcttttccacagatagtacactcatatggttttactccggcagtcttcttcgtcacactgagattgggactgaagttttctgcacattgactaccttctttaccttcacagagtctctctcccgtatggcttcttagatttcgtccttggtttttgtgttgatcttcaacattcgggtcttcccatttttcccctatagatgccaggttcttgaatgtttcctgcatcacatctctgtagagtttcttctgtgaaggagccagcagagcccactcctcctggctgaagctcacagacacatcctcaaaagccactgagtctattgctttcagaaaatgagaatgttgggccggtaatagtagctcatgcctggaatcctagcactttgggatgctgagggtggaggatcgcttgagcccaggagttcaagatcagcctgagcaacacagccagac

SEQ ID NO: 13872 - RNA, 2267 nt, Homo sapiens
  source 1..2267: mol_type = other RNA
gctgggattacaggcatgagccaccatgctcagcctaacagtgcctttaaaaacctcctgggctacattgaaaaccttattatcacatgtcaacttattttgaagcaagtttgcttataatttagtaaagtccttgtaaaacttcttgtttctctccactgtcactcagttttctgaaaactttaagtagaagcaaggccttggcaacaagataactcatcacatggttcaaagtatatctgtgcaatggatcaaatttacctattatcttgcacactgctctcagttataacctgagaaccagaaattatcccctcactttataaaaataccgttttaaaagattatttaacagcataatctttttaaatcaatgtgtaatactgaaaaacactatacatgtattttatctctctggggttaaaaaaaagtctgaggtgtactgaagggtactttctgttgcttcttcagatcttgtatattaacatttaagcacaaataccctttgtcaagtgctttcaatgccagaatctgtgcttattcaaaaatgaaaacaaaacaaccaaataattaatagtctctgcagaccaaagcgtaaatggattaacaaataacactgaatgcaaattcaggtaaccatatcaaaccaagaggaaagaatgtggttcatcttttggaggagttgtctaaaaggatccaatcaatcacaacctctctttttctctgcaatgatacaccagttaccatgatcattcccagaactcaggatacggagctctgacacattctccttgagcagactgcagagctccccttctcgaaacacatggtagtagcgcataaaggctgtggagtccaaaacatcagtctgtggatcttcgacagacattgtatcatctgggttgaaatctgtggaatcaactgcagaaatccttctcaatattttactagcagaaggattatcatcttctatgttgcctgcatccacacaattcacaccagtattagtgctatccagaaaatttccccctccatttctcctcatttccccttgatggtctccatttaaatgtttcagagtgcctggtgctctcagccactccaagtgttttccagaagaagattccacaaacacttcctcatctaaactttgcccttttgttgaaaatggctcttggtgatcaaagtctaaactagagtgtctggaaggctggactgttacagtgctactggcccaaacttctgtgtttttcaagggtcttactctttcaatttgcttcctcagagtcgattcatccaaagatctggagaaaaaccaggaacgaaacgattttcctaatgtgctgtaaaatccatattcttcctcgccttccttagaaatatttgcaaaacaggttcttgccatagcaggttcatagcccacgctgtgggaccgttttgaaccacactgctctttaaaacaaacagaacagctacactcagagcaaggaggatggtagggatggcctctttctgggtatccacactgcctcttcctcccagactggctggactctgagaagagctgggaacacagagccctgttccatggaacaagcacgtcttgcttctcaaagtgacggttcttttgttccattgcccaaacgtaaatcatcagttggcctccgggaactaagaccctggccatttcttttattgctctgattcttctttgttttgtagaaaaatgatgtatgacatggcttcacatcctctattccgggcaatctctaccagtggcccacagtagtcacagcccacggtatgtacctggctgttcactttaagatattttccagtcccacaacctataagagaaaaacctgcgttacatgctatcctcaatggaaaatgtgaaatacttcatttgtctcataacaagaaatataattaaccttttatttatttatttattttgagacagagtctccctcagtcacccaggctggagtgcagtggcgcaatctcggttcactgcaacctctgcctcacgggttcaagcaattctcttgccttagcctcccgagtaggtgggatcataggcgcgtgccaccatgaccggataattttgtatttttagtagagacgggtttctccatgttggtcaggttggtctcgaactcccaacctcaggtgatccgcctgcctcggcctcccaaagtgctgggattacaggtgcaagccactgtgcctggccaactttttttttttttttaactaaccaagac

SEQ ID NO: 13873 - RNA, 3200 nt, Homo sapiens
  source 1..3200: mol_type = other RNA
gctgggattacaggcatgagccaccatgctcagcctaacagtgcctttaaaaacctcctgggctacattgaaaaccttattatcacatgtcaacttattttgaagcaagtttgcttataatttagtaaagtccttgtaaaacttcttgtttctctccactgtcactcagttttctgaaaactttaagtagaagcaaggccttggcaacaagataactcatcacatggttcaaagtatatctgtgcaatggatcaaatttacctattatcttgcacactgctctcagttataacctgagaaccagaaattatcccctcactttataaaaataccgttttaaaagattatttaacagcataatctttttaaatcaatgtgtaatactgaaaaacactatacatgtattttatctctctggggttaaaaaaaagtctgaggtgtactgaagggtactttctgttgcttcttcagatcttgtatattaacatttaagcacaaataccctttgtcaagtgctttcaatgccagaatctgtgcttattcaaaaatgaaaacaaaacaaccaaataattaatagtctctgcagaccaaagcgtaaatggattaacaaataacactgaatgcaaattcaggtaaccatatcaaaccaagaggaaagaatgtggttcatcttttggaggagttgtctaaaaggatccaatcaatcacaacctctctttttctctgcaatgatacaccagttaccatgatcattcccagaactcaggatacggagctctgacacattctccttgagcagactgcagagctccccttctcgaaacacatggtagtagcgcataaaggctgtggagtccaaaacatcagtctgtggatcttcgacagacattgtatcatctgggttgaaatctgtggaatcaactgcagaaatccttctcaatattttactagcagaaggattatcatcttctatgttgcctgcatccacacaattcacaccagtattagtgctatccagaaaatttccccctccatttctcctcatttccccttgatggtctccatttaaatgtttcagagtgcctggtgctctcagccactccaagtgttttccagaagaagattccacaaacacttcctcatctaaactttgcccttttgttgaaaatggctcttggtgatcaaagtctaaactagagtgtctggaaggctggactgttacagtgctactggcccaaacttctgtgtttttcaagggtcttactctttcaatttgcttcctcagagtcgattcatccaaagatctggagaaaaaccaggaacgaaacgattttcctaatgtgctgtaaaatccatattcttcctcgccttccttagaaatatttgcaaaacaggttcttgccatagcaggttcatagcccacgctgtgggaccgttttgaaccacactgctctttaaaacaaacagaacagctacactcagagcaaggaggatggtagggatggcctctttctgggtatccacactgcctcttcctcccagactggctggactctgagaagagctgggaacacagagccctgttccatggaacaagcacgtcttgcttctcaaagtgacggttcttttgttccattgcccaaacgtaaatcatcagttggcctccgggaactaagaccctggccatttcttttattgctctgattcttctttgttttgtagaaaaatgatgtatgacatggcttcacatcctctattccgggcaatctctaccagtggcccacagtagtcacagcccacggtatgtacctggctgttcactttaagatattttccagtcccacaacctataagagaaaaacctgcgttacatgctatcctcaatggaaaatgtgaaatacttcatttgtctcataacaagaaatataattaaccttttatttatttatttattttgagacagagtctccctcagtcacccaggctggagtgcagtggcgcaatctcggttcactgcaacctctgcctcacgggttcaagcaattctcttgccttagcctcccgagtaggtgggatcataggcgcgtgccaccatgaccggataattttgtatttttagtagagacgggtttctccatgttggtcaggttggtctcgaactcccaacctcaggtgatccgcctgcctcggcctcccaaagtgctgggattacaggtgcaagccactgtgcctggccaactttttttttttttttaactaaccaagacagaatacaacatggtgtgaaggtattcacaaaagcaaaagaaaagccttcggcgaatacttacagattctcatatagaagagagaaaggcaataggaaaaaaataacatttattgaatatttaatgaggtgatgtccacagggctcagtacactggcgcaaccaaggcacgttagctggtccaaggcaagaaagatagttctagtatccgagagaccacgtgtagcctctaagctcacattcatatttcattttgtatatacgcatgtttcggcttttattctcctgttgtctctccaaagattcttaccacttgctgactgagtcatcctgtgattacaggaaaattacctcttgtctttgtgaatcacggcagtctccacctccagagagtgacagttgcttctcataactttctcaatgtgtaacgtaaatgaaaacttgtaggagtgaaatgaaatagtgcggtccttctcatgataaacctcttgtgtgagtctctgaaggaagcacaggccccaggcggccagacccgggcgcgggctccggggcacgcgctagacgacctgtcgcgccccctcctccctgcgggcgggcgccgaggcagcggatctagggcgcaacagaagcttctctccgctcccctatgcagaccattgtcagtgctccggtcgccggcgctttccgcacggtgtggcgactggcagcagctctcccgttgcgagtagtcacagcgctgtcccgcagccaggggcaaaagctgcttttgcatcagagccgagggctgcaccaggtgtaacttccaccccttgacctattttagagtgtgaggatgaaaggaagaggaaaaaatagacggagggcgcgcgggggtgcgggcggcagggtgcgcgcgtggccgtgggggagcgcgcgcgcgggccggggctcgtgt

SEQ ID NO: 13874 - RNA, 2257 nt, Homo sapiens
  source 1..2257: mol_type = other RNA
gctgggattacaggcatgagccaccatgctcagcctaacagtgcctttaaaaacctcctgggctacattgaaaaccttattatcacatgtcaacttattttgaagcaagtttgcttataatttagtaaagtccttgtaaaacttcttgtttctctccactgtcactcagttttctgaaaactttaagtagaagcaaggccttggcaacaagataactcatcacatggttcaaagtatatctgtgcaatggatcaaatttacctattatcttgcacactgctctcagttataacctgagaaccagaaattatcccctcactttataaaaataccgttttaaaagattatttaacagcataatctttttaaatcaatgtgtaatactgaaaaacactatacatgtattttatctctctggggttaaaaaaaagtctgaggtgtactgaagggtactttctgttgcttcttcagatcttgtatattaacatttaagcacaaataccctttgtcaagtgctttcaatgccagaatctgtgcttattcaaaaatgaaaacaaaacaaccaaataattaatagtctctgcagaccaaagcgtaaatggattaacaaataacactgaatgcaaattcaggtaaccatatcaaaccaagaggaaagaatgtggttcatcttttggaggagttgtctaaaaggatccaatcaatcacaacctctctttttctctgcaatgatacaccagttaccatgatcattcccagaactcaggatacggagctctgacacattctccttgagcagactgcagagctccccttctcgaaacacatggtagtagcgcataaaggctgtggagtccaaaacatcagtctgtggatcttcgacagacattgtatcatctgggttgaaatctgtggaatcaactgcagaaatccttctcaatattttactagcagaaggattatcatcttctatgttgcctgcatccacacaattcacaccagtattagtgctatccagaaaatttccccctccatttctcctcatttccccttgatggtctccatttaaatgtttcagagtgcctggtgctctcagccactccaagtgttttccagaagaagattccacaaacacttcctcatctaaactttgcccttttgttgaaaatggctcttggtgatcaaagtctaaactagagtgtctggaaggctggactgttacagtgctactggcccaaacttctgtgtttttcaagggtcttactctttcaatttgcttcctcagagtcgattcatccaaagatctggagaaaaaccaggaacgaaacgattttcctaatgtgctgtaaaatccatattcttcctcgccttccttagaaatatttgcaaaacaggttcttgccatagcaggttcatagcccacgctgtgggaccgttttgaaccacactgctctttaaaacaaacagaacagctacactcagagcaaggaggatggtagggatggcctctttctgggtatccacactgcctcttcctcccagactggctggactctgagaagagctgggaacacagagccctgttccatggaacaagcacgtcttgcttctcaaagtgacggttcttttgttccattgcccaaacgtaaatcatcagttggcctccgggaactaagaccctggccatttcttttattgctctgattcttctttgttttgtagaaaaatgatgtatgactcctatggagatgatggcatcgaagccctcatccctaaaggggagattaaggttgtcacataccatggcttcacatcctctattccgggcaatctctaccagtggcccacagtagtcacagcccacggtatgtacctggctgttcactttaagatattttccagtcccacaacagattctcatatagaagagagaaaggcaataggaaaaaaataacatttattgaatatttaatgaggtgatgtccacagggctcagtacactggcgcaaccaaggcacgttagctggtccaaggcaagaaagatagttctagtatccgagagaccacgtgtagcctctaagctcacattcatatttcattttgtatatacgcatgtttcggcttttattctcctgttgtctctccaaagattcttaccacttgctgactatgtcagcgatgaggctgcctggcttctgctcttgcaggaactggcggacacgaggccaggctttgctctgcaggtcgctgaagtaag

SEQ ID NO: 13875 - RNA, 2361 nt, Homo sapiens
  source 1..2361: mol_type = other RNA
gctgggattacaggcatgagccaccatgctcagcctaacagtgcctttaaaaacctcctgggctacattgaaaaccttattatcacatgtcaacttattttgaagcaagtttgcttataatttagtaaagtccttgtaaaacttcttgtttctctccactgtcactcagttttctgaaaactttaagtagaagcaaggccttggcaacaagataactcatcacatggttcaaagtatatctgtgcaatggatcaaatttacctattatcttgcacactgctctcagttataacctgagaaccagaaattatcccctcactttataaaaataccgttttaaaagattatttaacagcataatctttttaaatcaatgtgtaatactgaaaaacactatacatgtattttatctctctggggttaaaaaaaagtctgaggtgtactgaagggtactttctgttgcttcttcagatcttgtatattaacatttaagcacaaataccctttgtcaagtgctttcaatgccagaatctgtgcttattcaaaaatgaaaacaaaacaaccaaataattaatagtctctgcagaccaaagcgtaaatggattaacaaataacactgaatgcaaattcaggtaaccatatcaaaccaagaggaaagaatgtggttcatcttttggaggagttgtctaaaaggatccaatcaatcacaacctctctttttctctgcaatgatacaccagttaccatgatcattcccagaactcaggatacggagctctgacacattctccttgagcagactgcagagctccccttctcgaaacacatggtagtagcgcataaaggctgtggagtccaaaacatcagtctgtggatcttcgacagacattgtatcatctgggttgaaatctgtggaatcaactgcagaaatccttctcaatattttactagcagaaggattatcatcttctatgttgcctgcatccacacaattcacaccagtattagtgctatccagaaaatttccccctccatttctcctcatttccccttgatggtctccatttaaatgtttcagagtgcctggtgctctcagccactccaagtgttttccagaagaagattccacaaacacttcctcatctaaactttgcccttttgttgaaaatggctcttggtgatcaaagtctaaactagagtgtctggaaggctggactgttacagtgctactggcccaaacttctgtgtttttcaagggtcttactctttcaatttgcttcctcagagtcgattcatccaaagatctggagaaaaaccaggaacgaaacgattttcctaatgtgctgtaaaatccatattcttcctcgccttccttagaaatatttgcaaaacaggttcttgccatagcaggttcatagcccacgctgtgggaccgttttgaaccacactgctctttaaaacaaacagaacagctacactcagagcaaggaggatggtagggatggcctctttctgggtatccacactgcctcttcctcccagactggctggactctgagaagagctgggaacacagagccctgttccatggaacaagcacgtcttgcttctcaaagtgacggttcttttgttccattgcccaaacgtaaatcatcagttggcctccgggaactaagaccctggccatttcttttattgctctgattcttctttgttttgtagaaaaatgatgtatgactcctatggagatgatggcatcgaagccctcatccctaaaggggagattaaggttgtcacataccatggcttcacatcctctattccgggcaatctctaccagtggcccacagtagtcacagcccacggtatgtacctggctgttcactttaagatattttccagtcccacaacagattctcatatagaagagagaaaggcaataggaaaaaaataacatttattgaatatttaatgaggtgatgtccacagggctcagtacactggcgcaaccaaggcacgttagctggtccaaggcaagaaagatagttctagtatccgagagaccacgtgtagcctctaagctcacattcatatttcattttgtatatacgcatgtttcggcttttattctcctgttgtctctccaaagattcttaccacttgctgactatgtcagcgatgaggctgcctggttacctatgtcagcgatgaggctgcctggttacctatgtcagcgatgaggctgcctggttacctatgtcagcgatgaggctgcctggcttctgctcttgcaggaactggcggacacgaggccaggctttgctctgcaggtcgctgaagtaaggggctgtgctctcgtac

SEQ ID NO: 13876 - RNA, 2781 nt, Homo sapiens
  source 1..2781: mol_type = other RNA
gctgggattacaggcatgagccaccatgctcagcctaacagtgcctttaaaaacctcctgggctacattgaaaaccttattatcacatgtcaacttattttgaagcaagtttgcttataatttagtaaagtccttgtaaaacttcttgtttctctccactgtcactcagttttctgaaaactttaagtagaagcaaggccttggcaacaagataactcatcacatggttcaaagtatatctgtgcaatggatcaaatttacctattatcttgcacactgctctcagttataacctgagaaccagaaattatcccctcactttataaaaataccgttttaaaagattatttaacagcataatctttttaaatcaatgtgtaatactgaaaaacactatacatgtattttatctctctggggttaaaaaaaagtctgaggtgtactgaagggtactttctgttgcttcttcagatcttgtatattaacatttaagcacaaataccctttgtcaagtgctttcaatgccagaatctgtgcttattcaaaaatgaaaacaaaacaaccaaataattaatagtctctgcagaccaaagcgtaaatggattaacaaataacactgaatgcaaattcaggtaaccatatcaaaccaagaggaaagaatgtggttcatcttttggaggagttgtctaaaaggatccaatcaatcacaacctctctttttctctgcaatgatacaccagttaccatgatcattcccagaactcaggatacggagctctgacacattctccttgagcagactgcagagctccccttctcgaaacacatggtagtagcgcataaaggctgtggagtccaaaacatcagtctgtggatcttcgacagacattgtatcatctgggttgaaatctgtggaatcaactgcagaaatccttctcaatattttactagcagaaggattatcatcttctatgttgcctgcatccacacaattcacaccagtattagtgctatccagaaaatttccccctccatttctcctcatttccccttgatggtctccatttaaatgtttcagagtgcctggtgctctcagccactccaagtgttttccagaagaagattccacaaacacttcctcatctaaactttgcccttttgttgaaaatggctcttggtgatcaaagtctaaactagagtgtctggaaggctggactgttacagtgctactggcccaaacttctgtgtttttcaagggtcttactctttcaatttgcttcctcagagtcgattcatccaaagatctggagaaaaaccaggaacgaaacgattttcctaatgtgctgtaaaatccatattcttcctcgccttccttagaaatatttgcaaaacaggttcttgccatagcaggttcatagcccacgctgtgggaccgttttgaaccacactgctctttaaaacaaacagaacagctacactcagagcaaggaggatggtagggatggcctctttctgggtatccacactgcctcttcctcccagactggctggactctgagaagagctgggaacacagagccctgttccatggaacaagcacgtcttgcttctcaaagtgacggttcttttgttccattgcccaaacgtaaatcatcagttggcctccgggaactaagaccctggccatttcttttattgctctgattcttctttgttttgtagaaaaatgatgtatgactcctatggagatgatggcatcgaagccctcatccctaaaggggagattaaggttgtcacataccatggcttcacatcctctattccgggcaatctctaccagtggcccacagtagtcacagcccacggtatgtacctggctgttcactttaagatattttccagtcccacaacagattctcatatagaagagagaaaggcaataggaaaaaaataacatttattgaatatttaatgaggtgatgtccacagggctcagtacactggcgcaaccaaggcacgttagctggtccaaggcaagaaagatagttctagtatccgagagaccacgtgtagcctctaagctcacattcatatttcattttgtatatacgcatgtttcggcttttattctcctgttgtctctccaaagattcttaccacttgctgactgagtcatcctgtgattacaggaaaattacctcttgtctttgtgaatcacggcagtctccacctccagagagtgacagttgcttctcataactttctcaatgtgtaacgtaaatgaaaacttgtaggagtgaaatgaaatagtgcggtccttctcatgataaacctcttgtgtgagtctctgaaggaagcacaggccccaggcggccagacccgggcgcgggctccggggcacgcgctagacgacctgtcgcgccccctcctccctgcgggcgggcgccgaggcagcggatctagggcgcaacagaagcttctctccgctcccctatgcagaccattgtcagtgctccggtcgccggcgctttccgcacggtgtggcgactggcagcagctctcccgttgcgagtagtcacagcgctgtcccgcagccaggggcaaaagctgcttttgcatcagagccgagggctgcaccaggtgtaacttccaccccttgacctattttagagtgtgaggatgaaaggaagaggaaaaaatagacggagggcgcgcgggggtgcgggcggcagggtgcgcgcgtggccgtgggggagcgcgcgcgcgggccggggctcgtgt

SEQ ID NO: 13877 - RNA, 3120 nt, Homo sapiens
  source 1..3120: mol_type = other RNA
gctgggattacaggcatgagccaccatgctcagcctaacagtgcctttaaaaacctcctgggctacattgaaaaccttattatcacatgtcaacttattttgaagcaagtttgcttataatttagtaaagtccttgtaaaacttcttgtttctctccactgtcactcagttttctgaaaactttaagtagaagcaaggccttggcaacaagataactcatcacatggttcaaagtatatctgtgcaatggatcaaatttacctattatcttgcacactgctctcagttataacctgagaaccagaaattatcccctcactttataaaaataccgttttaaaagattatttaacagcataatctttttaaatcaatgtgtaatactgaaaaacactatacatgtattttatctctctggggttaaaaaaaagtctgaggtgtactgaagggtactttctgttgcttcttcagatcttgtatattaacatttaagcacaaataccctttgtcaagtgctttcaatgccagaatctgtgcttattcaaaaatgaaaacaaaacaaccaaataattaatagtctctgcagaccaaagcgtaaatggattaacaaataacactgaatgcaaattcaggtaaccatatcaaaccaagaggaaagaatgtggttcatcttttggaggagttgtctaaaaggatccaatcaatcacaacctctctttttctctgcaatgatacaccagttaccatgatcattcccagaactcaggatacggagctctgacacattctccttgagcagactgcagagctccccttctcgaaacacatggtagtagcgcataaaggctgtggagtccaaaacatcagtctgtggatcttcgacagacattgtatcatctgggttgaaatctgtggaatcaactgcagaaatccttctcaatattttactagcagaaggattatcatcttctatgttgcctgcatccacacaattcacaccagtattagtgctatccagaaaatttccccctccatttctcctcatttccccttgatggtctccatttaaatgtttcagagtgcctggtgctctcagccactccaagtgttttccagaagaagattccacaaacacttcctcatctaaactttgcccttttgttgaaaatggctcttggtgatcaaagtctaaactagagtgtctggaaggctggactgttacagtgctactggcccaaacttctgtgtttttcaagggtcttactctttcaatttgcttcctcagagtcgattcatccaaagatctggagaaaaaccaggaacgaaacgattttcctaatgtgctgtaaaatccatattcttcctcgccttccttagaaatatttgcaaaacaggttcttgccatagcaggttcatagcccacgctgtgggaccgttttgaaccacactgctctttaaaacaaacagaacagctacactcagagcaaggaggatggtagggatggcctctttctgggtatccacactgcctcttcctcccagactggctggactctgagaagagctgggaacacagagccctgttccatggaacaagcacgtcttgcttctcaaagtgacggttcttttgttccattgcccaaacgtaaatcatcagttggcctccgggaactaagaccctggccatttcttttattgctctgattcttctttgttttgtagaaaaatgatgtatgactcctatggagatgatggcatcgaagccctcatccctaaaggggagattaaggttgtcacataccatggcttcacatcctctattccgggcaatctctaccagtggcccacagtagtcacagcccacggtatgtacctggctgttcactttaagatattttccagtcccacaacctatgtcagcgatgaggctgcctggcttctgctcttgcaggaactggcggacacgaggccaggctttgctctgcaggtcgctgaagtaaggggctgtgctctcgtacacattgtgcacatgctgcttctccagctgggcggcttcatgatccatcccaggcggccagacccgggcgcgggctccggggcacgcgctagacgacctgtcgcgccccctcctccctgcgggcgggcgccgaggcagcggatctagggcgcaacagaagcttctctccgctcccctatgcagaccattgtcagtgctccggtcgccggcgctttccgcacggtgtggcgactggcagcagctctcccgttgcgagtagtcacagcgctgtcccgcagccaggggcaaaagctgcttttgcatcagagccgagggctgcaccaggtgtaacttccaccccttgaccttgggtgacgacgacgcttggctttagcgcggctcttctcacttaattttttacagccccggacttcagcggaaatgccccctcggggtcggttcattgggataactggagatgggggggttaagtagggtgccacggcttagacgctccaaatcattccactacacaacatgcctaatctgctgagttttgcaaaacgagccccatcaaaaaagcatccatcagaaggcggggtggaacttagaagtttttgcccaaaactggacacaaacctttcctccccccattgcttctatgacaatagcgttaactactttcttccaggtccctaacgtaatagtatcttcaaccgcctattatcaaacaactccgttatcatcagggatctatgcactttaaaaatgcacgttcttagtgacgaaaaatgagcacatttagtaaccgctctgccgccctttgtatagaggttcgtgctcctgatccccagcgtagggggcagagttcatgtcgagctgttgtttccagttcaggttatttatggggacccaactacaggtctcacatagacgctggtctataacaggttatttgtgaggacacaactacaggtctcacatagacgctggtctatttcaggtgctactaagagggctaatggacgtcagcatatagtttctgattctggaatcgttttctagtgccacagtatattgggtggggtggagtgggggaaacctttgtttgggcttctctttat

SEQ ID NO: 13878 - RNA, 2443 nt, Homo sapiens
  source 1..2443: mol_type = other RNA
gctgggattacaggcatgagccaccatgctcagcctaacagtgcctttaaaaacctcctgggctacattgaaaaccttattatcacatgtcaacttattttgaagcaagtttgcttataatttagtaaagtccttgtaaaacttcttgtttctctccactgtcactcagttttctgaaaactttaagtagaagcaaggccttggcaacaagataactcatcacatggttcaaagtatatctgtgcaatggatcaaatttacctattatcttgcacactgctctcagttataacctgagaaccagaaattatcccctcactttataaaaataccgttttaaaagattatttaacagcataatctttttaaatcaatgtgtaatactgaaaaacactatacatgtattttatctctctggggttaaaaaaaagtctgaggtgtactgaagggtactttctgttgcttcttcagatcttgtatattaacatttaagcacaaataccctttgtcaagtgctttcaatgccagaatctgtgcttattcaaaaatgaaaacaaaacaaccaaataattaatagtctctgcagaccaaagcgtaaatggattaacaaataacactgaatgcaaattcaggtaaccatatcaaaccaagaggaaagaatgtggttcatcttttggaggagttgtctaaaaggatccaatcaatcacaacctctctttttctctgcaatgatacaccagttaccatgatcattcccagaactcaggatacggagctctgacacattctccttgagcagactgcagagctccccttctcgaaacacatggtagtagcgcataaaggctgtggagtccaaaacatcagtctgtggatcttcgacagacattgtatcatctgggttgaaatctgtggaatcaactgcagaaatccttctcaatattttactagcagaaggattatcatcttctatgttgcctgcatccacacaattcacaccagtattagtgctatccagaaaatttccccctccatttctcctcatttccccttgatggtctccatttaaatgtttcagagtgcctggtgctctcagccactccaagtgttttccagaagaagattccacaaacacttcctcatctaaactttgcccttttgttgaaaatggctcttggtgatcaaagtctaaactagagtgtctggaaggctggactgttacagtgctactggcccaaacttctgtgtttttcaagggtcttactctttcaatttgcttcctcagagtcgattcatccaaagatctggagaaaaaccaggaacgaaacgattttcctaatgtgctgtaaaatccatattcttcctcgccttccttagaaatatttgcaaaacaggttcttgccatagcaggttcatagcccacgctgtgggaccgttttgaaccacactgctctttaaaacaaacagaacagctacactcagagcaaggaggatggtagggatggcctctttctgggtatccacactgcctcttcctcccagactggctggactctgagaagagctgggaacacagagccctgttccatggaacaagcacgtcttgcttctcaaagtgacggttcttttgttccattgcccaaacgtaaatcatcagttggcctccgggaactaagaccctggccatttcttttattgctctgattcttctttgttttgtagaaaaatgatgtatgactcctatggagatgatggcatcgaagccctcatccctaaaggggagattaaggttgtcacataccatggcttcacatcctctattccgggcaatctctaccagtggcccacagtagtcacagcccacggtatgtacctggctgttcactttaagatattttccagtcccacaacctatgtcagcgatgaggctgcctggcttctgctcttgcaggaactggcggacacgaggccaggctttgctctgcaggtcgctgaagtaaggggctgtgctctcgtacacattgtgcacatgctgcttctccagctgggcggcttcatgatccatcccaggcggccagacccgggcgcgggctccggggcacgcgctagacgacctgtcgcgccccctcctccctgcgggcgggcgccgaggcagcggatctagggcgcaacagaagcttctctccgctcccctatgcagaccattgtcagtgctccggtcgccggcgctttccgcacggtgtggcgactggcagcagctctcccgttgcgagtagtcacagcgctgtcccgcagccaggggcaaaagctgcttttgcatcagagccgagggctgcaccaggtgtaacttccaccccttgacctttcgggaggcggcgctcgggctcagctgtccgggaacccaggcctgcggcgcctccgggcagcgaaggcgggctggcgc

SEQ ID NO: 13879 - RNA, 2649 nt, Homo sapiens
  source 1..2649: mol_type = other RNA
gctgggattacaggcatgagccaccatgctcagcctaacagtgcctttaaaaacctcctgggctacattgaaaaccttattatcacatgtcaacttattttgaagcaagtttgcttataatttagtaaagtccttgtaaaacttcttgtttctctccactgtcactcagttttctgaaaactttaagtagaagcaaggccttggcaacaagataactcatcacatggttcaaagtatatctgtgcaatggatcaaatttacctattatcttgcacactgctctcagttataacctgagaaccagaaattatcccctcactttataaaaataccgttttaaaagattatttaacagcataatctttttaaatcaatgtgtaatactgaaaaacactatacatgtattttatctctctggggttaaaaaaaagtctgaggtgtactgaagggtactttctgttgcttcttcagatcttgtatattaacatttaagcacaaataccctttgtcaagtgctttcaatgccagaatctgtgcttattcaaaaatgaaaacaaaacaaccaaataattaatagtctctgcagaccaaagcgtaaatggattaacaaataacactgaatgcaaattcaggtaaccatatcaaaccaagaggaaagaatgtggttcatcttttggaggagttgtctaaaaggatccaatcaatcacaacctctctttttctctgcaatgatacaccagttaccatgatcattcccagaactcaggatacggagctctgacacattctccttgagcagactgcagagctccccttctcgaaacacatggtagtagcgcataaaggctgtggagtccaaaacatcagtctgtggatcttcgacagacattgtatcatctgggttgaaatctgtggaatcaactgcagaaatccttctcaatattttactagcagaaggattatcatcttctatgttgcctgcatccacacaattcacaccagtattagtgctatccagaaaatttccccctccatttctcctcatttccccttgatggtctccatttaaatgtttcagagtgcctggtgctctcagccactccaagtgttttccagaagaagattccacaaacacttcctcatctaaactttgcccttttgttgaaaatggctcttggtgatcaaagtctaaactagagtgtctggaaggctggactgttacagtgctactggcccaaacttctgtgtttttcaagggtcttactctttcaatttgcttcctcagagtcgattcatccaaagatctggagaaaaaccaggaacgaaacgattttcctaatgtgctgtaaaatccatattcttcctcgccttccttagaaatatttgcaaaacaggttcttgccatagcaggttcatagcccacgctgtgggaccgttttgaaccacactgctctttaaaacaaacagaacagctacactcagagcaaggaggatggtagggatggcctctttctgggtatccacactgcctcttcctcccagactggctggactctgagaagagctgggaacacagagccctgttccatggaacaagcacgtcttgcttctcaaagtgacggttcttttgttccattgcccaaacgtaaatcatcagttggcctccgggaactaagaccctggccatttcttttattgctctgattcttctttgttttgtagaaaaatgatgtatgactcctatggagatgatggcatcgaagccctcatccctaaaggggagattaaggttgtcacataccatggcttcacatcctctattccgggcaatctctaccagtggcccacagtagtcacagcccacggtatgtacctggctgttcactttaagatattttccagtcccacaacctatgtcagcgatgaggctgcctggcttctgctcttgcaggaactggcggacacgaggccaggctttgctctgcaggtcgctgaagtaaggggctgtgctctcgtacacattgtgcacatgctgcttctccagctgggcggcttcatgatccatcctcttgtctttgtgaatcacggcagtctccacctccagagagtgacagttgcttctcataactttctcaatgtgtaacgtaaatgaaaacttgtaggagtgaaatgaaatagtgcggtccttctcatgataaacctcttgtgtgagtctctgaaggaagcacaggccccaggcggccagacccgggcgcgggctccggggcacgcgctagacgacctgtcgcgccccctcctccctgcgggcgggcgccgaggcagcggatctagggcgcaacagaagcttctctccgctcccctatgcagaccattgtcagtgctccggtcgccggcgctttccgcacggtgtggcgactggcagcagctctcccgttgcgagtagtcacagcgctgtcccgcagccaggggcaaaagctgcttttgcatcagagccgagggctgcaccaggtgtaacttccaccccttgacctattttagagtgtgaggatgaaaggaagaggaaaaaatagacggagggcgcgcgggggtgcgggcggcagggtgcgcgcgtggccgtgggggagcgcgcgcgcgggccggggctcgtgt

SEQ ID NO: 13880 - RNA, 2579 nt, Homo sapiens
  source 1..2579: mol_type = other RNA
gctgggattacaggcatgagccaccatgctcagcctaacagtgcctttaaaaacctcctgggctacattgaaaaccttattatcacatgtcaacttattttgaagcaagtttgcttataatttagtaaagtccttgtaaaacttcttgtttctctccactgtcactcagttttctgaaaactttaagtagaagcaaggccttggcaacaagataactcatcacatggttcaaagtatatctgtgcaatggatcaaatttacctattatcttgcacactgctctcagttataacctgagaaccagaaattatcccctcactttataaaaataccgttttaaaagattatttaacagcataatctttttaaatcaatgtgtaatactgaaaaacactatacatgtattttatctctctggggttaaaaaaaagtctgaggtgtactgaagggtactttctgttgcttcttcagatcttgtatattaacatttaagcacaaataccctttgtcaagtgctttcaatgccagaatctgtgcttattcaaaaatgaaaacaaaacaaccaaataattaatagtctctgcagaccaaagcgtaaatggattaacaaataacactgaatgcaaattcaggtaaccatatcaaaccaagaggaaagaatgtggttcatcttttggaggagttgtctaaaaggatccaatcaatcacaacctctctttttctctgcaatgatacaccagttaccatgatcattcccagaactcaggatacggagctctgacacattctccttgagcagactgcagagctccccttctcgaaacacatggtagtagcgcataaaggctgtggagtccaaaacatcagtctgtggatcttcgacagacattgtatcatctgggttgaaatctgtggaatcaactgcagaaatccttctcaatattttactagcagaaggattatcatcttctatgttgcctgcatccacacaattcacaccagtattagtgctatccagaaaatttccccctccatttctcctcatttccccttgatggtctccatttaaatgtttcagagtgcctggtgctctcagccactccaagtgttttccagaagaagattccacaaacacttcctcatctaaactttgcccttttgttgaaaatggctcttggtgatcaaagtctaaactagagtgtctggaaggctggactgttacagtgctactggcccaaacttctgtgtttttcaagggtcttactctttcaatttgcttcctcagagtcgattcatccaaagatctggagaaaaaccaggaacgaaacgattttcctaatgtgctgtaaaatccatattcttcctcgccttccttagaaatatttgcaaaacaggttcttgccatagcaggttcatagcccacgctgtgggaccgttttgaaccacactgctctttaaaacaaacagaacagctacactcagagcaaggaggatggtagggatggcctctttctgggtatccacactgcctcttcctcccagactggctggactctgagaagagctgggaacacagagccctgttccatggaacaagcacgtcttgcttctcaaagtgacggttcttttgttccattgcccaaacgtaaatcatcagttggcctccgggaactaagaccctggccatttcttttattgctctgattcttctttgttttgtagaaaaatgatgtatgactcctatggagatgatggcatcgaagccctcatccctaaaggggagattaaggttgtcacataccatggcttcacatcctctattccgggcaatctctaccagtggcccacagtagtcacagcccacggtatgtacctggctgttcactttaagatattttccagtcccacaacctatgtcagcgatgaggctgcctggcttctgctcttgcaggaactggcggacacgaggccaggctttgctctgcaggtcgctgaagtaaggggctgtgctctcgtacacattgtgcacatgctgcttctccagctgggcggcttcatgatccatcctcttgtctttgtgaatcacggcagtctccacctccagagagtgacagttgcttctcataactttctcaatgtgtaacgtaaatgaaaacttgtaggagtgaaatgaaatagtgcggtccttctcatgataaacctcttgtgtgagtctctgaaggaagcacaggccccaggcggccagacccgggcgcgggctccggggcacgcgctagacgacctgtcgcgccccctcctccctgcgggcgggcgccgaggcagcggatctagggcgcaacagaagcttctctccgctcccctatgcagaccattgtcagtgctccggtcgccggcgctttccgcacggtgtggcgactggcagcagctctcccgttgcgagtagtcacagcgctgtcccgcagccaggggcaaaagctgcttttgcatcagagccgagggctgcaccaggtgtaacttccaccccttgaccttgggtgacgacgacgcttggctttagcgcggctcttctcacttaattt

SEQ ID NO: 13881 - RNA, 2440 nt, Homo sapiens
  source 1..2440: mol_type = other RNA
gctgggattacaggcatgagccaccatgctcagcctaacagtgcctttaaaaacctcctgggctacattgaaaaccttattatcacatgtcaacttattttgaagcaagtttgcttataatttagtaaagtccttgtaaaacttcttgtttctctccactgtcactcagttttctgaaaactttaagtagaagcaaggccttggcaacaagataactcatcacatggttcaaagtatatctgtgcaatggatcaaatttacctattatcttgcacactgctctcagttataacctgagaaccagaaattatcccctcactttataaaaataccgttttaaaagattatttaacagcataatctttttaaatcaatgtgtaatactgaaaaacactatacatgtattttatctctctggggttaaaaaaaagtctgaggtgtactgaagggtactttctgttgcttcttcagatcttgtatattaacatttaagcacaaataccctttgtcaagtgctttcaatgccagaatctgtgcttattcaaaaatgaaaacaaaacaaccaaataattaatagtctctgcagaccaaagcgtaaatggattaacaaataacactgaatgcaaattcaggtaaccatatcaaaccaagaggaaagaatgtggttcatcttttggaggagttgtctaaaaggatccaatcaatcacaacctctctttttctctgcaatgatacaccagttaccatgatcattcccagaactcaggatacggagctctgacacattctccttgagcagactgcagagctccccttctcgaaacacatggtagtagcgcataaaggctgtggagtccaaaacatcagtctgtggatcttcgacagacattgtatcatctgggttgaaatctgtggaatcaactgcagaaatccttctcaatattttactagcagaaggattatcatcttctatgttgcctgcatccacacaattcacaccagtattagtgctatccagaaaatttccccctccatttctcctcatttccccttgatggtctccatttaaatgtttcagagtgcctggtgctctcagccactccaagtgttttccagaagaagattccacaaacacttcctcatctaaactttgcccttttgttgaaaatggctcttggtgatcaaagtctaaactagagtgtctggaaggctggactgttacagtgctactggcccaaacttctgtgtttttcaagggtcttactctttcaatttgcttcctcagagtcgattcatccaaagatctggagaaaaaccaggaacgaaacgattttcctaatgtgctgtaaaatccatattcttcctcgccttccttagaaatatttgcaaaacaggttcttgccatagcaggttcatagcccacgctgtgggaccgttttgaaccacactgctctttaaaacaaacagaacagctacactcagagcaaggaggatggtagggatggcctctttctgggtatccacactgcctcttcctcccagactggctggactctgagaagagctgggaacacagagccctgttccatggaacaagcacgtcttgcttctcaaagtgacggttcttttgttccattgcccaaacgtaaatcatcagttggcctccgggaactaagaccctggccatttcttttattgctctgattcttctttgttttgtagaaaaatgatgtatgactcctatggagatgatggcatcgaagccctcatccctaaaggggagattaaggttgtcacataccatggcttcacatcctctattccgggcaatctctaccagtggcccacagtagtcacagcccacggtatgtacctggctgttcactttaagatattttccagtcccacaacctatgtcagcgatgaggctgcctggcttctgctcttgcaggaactggcggacacgaggccaggctttgctctgcaggtcgctgaagtaaggggctgtgctctcgtacacattgtgcacatgctgcttctccagctgggcggcttcatgatccatcctcttgtctttgtgaatcacggcagtctccacctccagagagtgacagttgcttctcataactttctcaatgtgtaacgtaaatgaaaacttgtaggagtgaaatgaaatagtgcggtccttctcatgataaacctcttgtgtgagtctctgaaggaagcacaggccctggaagaaaaccaggtggtattggtgttatcaccaggtgaggggctaaagtttattcagcaacagtgaggtcaccaaggatctccaaaagttctgcctcgttatgcatggttggccttctgtttctgagttccacacggaccaatctgaccaaccaggcggccagacccgggcgcgggctccggggcacgcgctagacgacctgtc

SEQ ID NO: 13882 - RNA, 2462 nt, Homo sapiens
  source 1..2462: mol_type = other RNA
gctgggattacaggcatgagccaccatgctcagcctaacagtgcctttaaaaacctcctgggctacattgaaaaccttattatcacatgtcaacttattttgaagcaagtttgcttataatttagtaaagtccttgtaaaacttcttgtttctctccactgtcactcagttttctgaaaactttaagtagaagcaaggccttggcaacaagataactcatcacatggttcaaagtatatctgtgcaatggatcaaatttacctattatcttgcacactgctctcagttataacctgagaaccagaaattatcccctcactttataaaaataccgttttaaaagattatttaacagcataatctttttaaatcaatgtgtaatactgaaaaacactatacatgtattttatctctctggggttaaaaaaaagtctgaggtgtactgaagggtactttctgttgcttcttcagatcttgtatattaacatttaagcacaaataccctttgtcaagtgctttcaatgccagaatctgtgcttattcaaaaatgaaaacaaaacaaccaaataattaatagtctctgcagaccaaagcgtaaatggattaacaaataacactgaatgcaaattcaggtaaccatatcaaaccaagaggaaagaatgtggttcatcttttggaggagttgtctaaaaggatccaatcaatcacaacctctctttttctctgcaatgatacaccagttaccatgatcattcccagaactcaggatacggagctctgacacattctccttgagcagactgcagagctccccttctcgaaacacatggtagtagcgcataaaggctgtggagtccaaaacatcagtctgtggatcttcgacagacattgtatcatctgggttgaaatctgtggaatcaactgcagaaatccttctcaatattttactagcagaaggattatcatcttctatgttgcctgcatccacacaattcacaccagtattagtgctatccagaaaatttccccctccatttctcctcatttccccttgatggtctccatttaaatgtttcagagtgcctggtgctctcagccactccaagtgttttccagaagaagattccacaaacacttcctcatctaaactttgcccttttgttgaaaatggctcttggtgatcaaagtctaaactagagtgtctggaaggctggactgttacagtgctactggcccaaacttctgtgtttttcaagggtcttactctttcaatttgcttcctcagagtcgattcatccaaagatctggagaaaaaccaggaacgaaacgattttcctaatgtgctgtaaaatccatattcttcctcgccttccttagaaatatttgcaaaacaggttcttgccatagcaggttcatagcccacgctgtgggaccgttttgaaccacactgctctttaaaacaaacagaacagctacactcagagcaaggaggatggtagggatggcctctttctgggtatccacactgcctcttcctcccagactggctggactctgagaagagctgggaacacagagccctgttccatggaacaagcacgtcttgcttctcaaagtgacggttcttttgttccattgcccaaacgtaaatcatcagttggcctccgggaactaagaccctggccatttcttttattgctctgattcttctttgttttgtagaaaaatgatgtatgactcctatggagatgatggcatcgaagccctcatccctaaaggggagattaaggttgtcacataccatggcttcacatcctctattccgggcaatctctaccagtggcccacagtagtcacagcccacggtatgtacctggctgttcactttaagatattttccagtcccacaacctatgtcagcgatgaggctgcctggcttctgctcttgcaggaactggcggacacgaggccaggctttgctctgcaggtcgctgaagtaaggggctgtgctctcgtacacattgtgcacatgctgcttctccagctgggcggcttcatgatccatcctcttgtctttgtgaatcacggcagtctccacctccagagagtgacagttgcttctcataactttctcaatgtgtaacgtaaatgaaaacttgtaggagtgaaatgaaatagtgcggtccttctcatgataaacctcttgtgtgagtctctgaaggaagcacaggccctggaagaaaaccaggtggtattggtgttatcaccaggtgaggggctaaagtttattcagcaacagtgaggtcaccaaggatctccaaaagttctgcctcgttatgcatggttggccttctgtttctgagttccacacggaccaatctgaccaactgtgtatcaaaaatatttaaaatcagaatcatgcctgtaattccagcattttgggaagctgaggtgggaggatg

SEQ ID NO: 13883 - RNA, 2573 nt, Homo sapiens
  source 1..2573: mol_type = other RNA
gctgggattacaggcatgagccaccatgctcagcctaacagtgcctttaaaaacctcctgggctacattgaaaaccttattatcacatgtcaacttattttgaagcaagtttgcttataatttagtaaagtccttgtaaaacttcttgtttctctccactgtcactcagttttctgaaaactttaagtagaagcaaggccttggcaacaagataactcatcacatggttcaaagtatatctgtgcaatggatcaaatttacctattatcttgcacactgctctcagttataacctgagaaccagaaattatcccctcactttataaaaataccgttttaaaagattatttaacagcataatctttttaaatcaatgtgtaatactgaaaaacactatacatgtattttatctctctggggttaaaaaaaagtctgaggtgtactgaagggtactttctgttgcttcttcagatcttgtatattaacatttaagcacaaataccctttgtcaagtgctttcaatgccagaatctgtgcttattcaaaaatgaaaacaaaacaaccaaataattaatagtctctgcagaccaaagcgtaaatggattaacaaataacactgaatgcaaattcaggtaaccatatcaaaccaagaggaaagaatgtggttcatcttttggaggagttgtctaaaaggatccaatcaatcacaacctctctttttctctgcaatgatacaccagttaccatgatcattcccagaactcaggatacggagctctgacacattctccttgagcagactgcagagctccccttctcgaaacacatggtagtagcgcataaaggctgtggagtccaaaacatcagtctgtggatcttcgacagacattgtatcatctgggttgaaatctgtggaatcaactgcagaaatccttctcaatattttactagcagaaggattatcatcttctatgttgcctgcatccacacaattcacaccagtattagtgctatccagaaaatttccccctccatttctcctcatttccccttgatggtctccatttaaatgtttcagagtgcctggtgctctcagccactccaagtgttttccagaagaagattccacaaacacttcctcatctaaactttgcccttttgttgaaaatggctcttggtgatcaaagtctaaactagagtgtctggaaggctggactgttacagtgctactggcccaaacttctgtgtttttcaagggtcttactctttcaatttgcttcctcagagtcgattcatccaaagatctggagaaaaaccaggaacgaaacgattttcctaatgtgctgtaaaatccatattcttcctcgccttccttagaaatatttgcaaaacaggttcttgccatagcaggttcatagcccacgctgtgggaccgttttgaaccacactgctctttaaaacaaacagaacagctacactcagagcaaggaggatggtagggatggcctctttctgggtatccacactgcctcttcctcccagactggctggactctgagaagagctgggaacacagagccctgttccatggaacaagcacgtcttgcttctcaaagtgacggttcttttgttccattgcccaaacgtaaatcatcagttggcctccgggaactaagaccctggccatttcttttattgctctgattcttctttgttttgtagaaaaatgatgtatgactcctatggagatgatggcatcgaagccctcatccctaaaggggagattaaggttgtcacataccatggcttcacatcctctattccgggcaatctctaccagtggcccacagtagtcacagcccacggtatgtacctggctgttcactttaagatattttccagtcccacaacctatgtcagcgatgaggctgcctggcttctgctcttgcaggaactggcggacacgaggccaggctttgctctgcaggtcgctgaagtaaggggctgtgctctcgtacacattgtgcacatgctgcttctccagctgggcggcttcatgatccatcctcttgtctttgtgaatcacggcagtctccacctccagagagtgacagttgcttctcataactttctcaatgtgtaacgtaaatgaaaacttgtaggagtgaaatgaaatagtgcggtccttctcatgataaacctcttgtgtgagtctctgaaggaagcacaggcccttcctattttggcattccttcttaaactgtattttcatcgtgagctttgaaaactttctggcttcaagttatcttagttctttgcctcttactaattaaaaatcagttccccagggaaagatacacgtgcactccatgaaaaaatacgaatccactttaacccttaaggcactagacatgtcctttatctctgaattctgatttatccaatctcacacccaaagcacatcccgcaatcccttactgcatggctgtctcgcctgttttgatcgtattgcaaggctgtttgcaaggtaaacagccaccccgggctactggaaaggcaggggacgagcagga

SEQ ID NO: 13884 - RNA, 2519 nt, Homo sapiens
  source 1..2519: mol_type = other RNA
gctgggattacaggcatgagccaccatgctcagcctaacagtgcctttaaaaacctcctgggctacattgaaaaccttattatcacatgtcaacttattttgaagcaagtttgcttataatttagtaaagtccttgtaaaacttcttgtttctctccactgtcactcagttttctgaaaactttaagtagaagcaaggccttggcaacaagataactcatcacatggttcaaagtatatctgtgcaatggatcaaatttacctattatcttgcacactgctctcagttataacctgagaaccagaaattatcccctcactttataaaaataccgttttaaaagattatttaacagcataatctttttaaatcaatgtgtaatactgaaaaacactatacatgtattttatctctctggggttaaaaaaaagtctgaggtgtactgaagggtactttctgttgcttcttcagatcttgtatattaacatttaagcacaaataccctttgtcaagtgctttcaatgccagaatctgtgcttattcaaaaatgaaaacaaaacaaccaaataattaatagtctctgcagaccaaagcgtaaatggattaacaaataacactgaatgcaaattcaggtaaccatatcaaaccaagaggaaagaatgtggttcatcttttggaggagttgtctaaaaggatccaatcaatcacaacctctctttttctctgcaatgatacaccagttaccatgatcattcccagaactcaggatacggagctctgacacattctccttgagcagactgcagagctccccttctcgaaacacatggtagtagcgcataaaggctgtggagtccaaaacatcagtctgtggatcttcgacagacattgtatcatctgggttgaaatctgtggaatcaactgcagaaatccttctcaatattttactagcagaaggattatcatcttctatgttgcctgcatccacacaattcacaccagtattagtgctatccagaaaatttccccctccatttctcctcatttccccttgatggtctccatttaaatgtttcagagtgcctggtgctctcagccactccaagtgttttccagaagaagattccacaaacacttcctcatctaaactttgcccttttgttgaaaatggctcttggtgatcaaagtctaaactagagtgtctggaaggctggactgttacagtgctactggcccaaacttctgtgtttttcaagggtcttactctttcaatttgcttcctcagagtcgattcatccaaagatctggagaaaaaccaggaacgaaacgattttcctaatgtgctgtaaaatccatattcttcctcgccttccttagaaatatttgcaaaacaggttcttgccatagcaggttcatagcccacgctgtgggaccgttttgaaccacactgctctttaaaacaaacagaacagctacactcagagcaaggaggatggtagggatggcctctttctgggtatccacactgcctcttcctcccagactggctggactctgagaagagctgggaacacagagccctgttccatggaacaagcacgtcttgcttctcaaagtgacggttcttttgttccattgcccaaacgtaaatcatcagttggcctccgggaactaagaccctggccatttcttttattgctctgattcttctttgttttgtagaaaaatgatgtatgactcctatggagatgatggcatcgaagccctcatccctaaaggggagattaaggttgtcacataccatggcttcacatcctctattccgggcaatctctaccagtggcccacagtagtcacagcccacggtatgtacctggctgttcactttaagatattttccagtcccacaacctatgtcagcgatgaggctgcctggcttctgctcttgcaggaactggcggacacgaggccaggctttgctctgcaggtcgctgaagtaaggggctgtgctctcgtacacattgtgcacatgctgcttctccagctgggcggcttcatgatccatcctcttgtctttgtgaatcacggcagtctccacctccagagagtgacagttgcttctcataactttctcaatgtgtaacgtaaatgaaaacttgtaggagtgaaatgaaatagtgcggtccttctcatgataaacctcttgtgtgagtctctgaaggaagcacaggcccttgaaggaagactgcagagttgctaggagagctcacaggtttcatcactttcccagagggaggactgtgtaggattcagccttagatcctgaaagtctagtccagagccctgcacatggaagtactgaataagttgaaggaacatatgcatcaagaaaaaaaattcaaaacaaactaacaaaaaacacaaaaaatgaaaaaagaataaaacaaagaaaaaaagccaaaagaacatgtgcatctacttctgacatatacatgtgtgatcttttctgtactacacaa

SEQ ID NO: 13885 - RNA, 2613 nt, Homo sapiens
  source 1..2613: mol_type = other RNA
gctgggattacaggcatgagccaccatgctcagcctaacagtgcctttaaaaacctcctgggctacattgaaaaccttattatcacatgtcaacttattttgaagcaagtttgcttataatttagtaaagtccttgtaaaacttcttgtttctctccactgtcactcagttttctgaaaactttaagtagaagcaaggccttggcaacaagataactcatcacatggttcaaagtatatctgtgcaatggatcaaatttacctattatcttgcacactgctctcagttataacctgagaaccagaaattatcccctcactttataaaaataccgttttaaaagattatttaacagcataatctttttaaatcaatgtgtaatactgaaaaacactatacatgtattttatctctctggggttaaaaaaaagtctgaggtgtactgaagggtactttctgttgcttcttcagatcttgtatattaacatttaagcacaaataccctttgtcaagtgctttcaatgccagaatctgtgcttattcaaaaatgaaaacaaaacaaccaaataattaatagtctctgcagaccaaagcgtaaatggattaacaaataacactgaatgcaaattcaggtaaccatatcaaaccaagaggaaagaatgtggttcatcttttggaggagttgtctaaaaggatccaatcaatcacaacctctctttttctctgcaatgatacaccagttaccatgatcattcccagaactcaggatacggagctctgacacattctccttgagcagactgcagagctccccttctcgaaacacatggtagtagcgcataaaggctgtggagtccaaaacatcagtctgtggatcttcgacagacattgtatcatctgggttgaaatctgtggaatcaactgcagaaatccttctcaatattttactagcagaaggattatcatcttctatgttgcctgcatccacacaattcacaccagtattagtgctatccagaaaatttccccctccatttctcctcatttccccttgatggtctccatttaaatgtttcagagtgcctggtgctctcagccactccaagtgttttccagaagaagattccacaaacacttcctcatctaaactttgcccttttgttgaaaatggctcttggtgatcaaagtctaaactagagtgtctggaaggctggactgttacagtgctactggcccaaacttctgtgtttttcaagggtcttactctttcaatttgcttcctcagagtcgattcatccaaagatctggagaaaaaccaggaacgaaacgattttcctaatgtgctgtaaaatccatattcttcctcgccttccttagaaatatttgcaaaacaggttcttgccatagcaggttcatagcccacgctgtgggaccgttttgaaccacactgctctttaaaacaaacagaacagctacactcagagcaaggaggatggtagggatggcctctttctgggtatccacactgcctcttcctcccagactggctggactctgagaagagctgggaacacagagccctgttccatggaacaagcacgtcttgcttctcaaagtgacggttcttttgttccattgcccaaacgtaaatcatcagttggcctccgggaactaagaccctggccatttcttttattgctctgattcttctttgttttgtagaaaaatgatgtatgactcctatggagatgatggcatcgaagccctcatccctaaaggggagattaaggttgtcacataccatggcttcacatcctctattccgggcaatctctaccagtggcccacagtagtcacagcccacggtatgtacctggctgttcactttaagatattttccagtcccacaacctatgtcagcgatgaggctgcctggcttctgctcttgcaggaactggcggacacgaggccaggctttgctctgcaggtcgctgaagtaaggggctgtgctctcgtacacattgtgcacatgctgcttctccagctgggcggcttcatgatccatcctgagtcatcctgtgattacaggaaaattacctcttgtctttgtgaatcacggcagtctccacctccagagagtgacagttgcttctcataactttctcaatgtgtaacgtaaatgaaaacttgtaggagtgaaatgaaatagtgcggtccttctcatgataaacctcttgtgtgagtctctgaaggaagcacaggccccaggcggccagacccgggcgcgggctccggggcacgcgctagacgacctgtcgcgccccctcctccctgcgggcgggcgccgaggcagcggatctagggcgcaacagaagcttctctccgctcccctatgcagaccattgtcagtgctccggtcgccggcgctttccgcacggtgtggcgactggcagcagctctcccgttgcgagtagtcacagcgctgtcccgcagccaggggcaaaagctgcttttgcatcagagccgagggctgcaccaggtgtaacttccaccccttgaccttgggtgacgacgacgcttggctttagcgcggctcttctcacttaatttttt

SEQ ID NO: 13886 - RNA, 2600 nt, Homo sapiens
  source 1..2600: mol_type = other RNA
gctgggattacaggcatgagccaccatgctcagcctaacagtgcctttaaaaacctcctgggctacattgaaaaccttattatcacatgtcaacttattttgaagcaagtttgcttataatttagtaaagtccttgtaaaacttcttgtttctctccactgtcactcagttttctgaaaactttaagtagaagcaaggccttggcaacaagataactcatcacatggttcaaagtatatctgtgcaatggatcaaatttacctattatcttgcacactgctctcagttataacctgagaaccagaaattatcccctcactttataaaaataccgttttaaaagattatttaacagcataatctttttaaatcaatgtgtaatactgaaaaacactatacatgtattttatctctctggggttaaaaaaaagtctgaggtgtactgaagggtactttctgttgcttcttcagatcttgtatattaacatttaagcacaaataccctttgtcaagtgctttcaatgccagaatctgtgcttattcaaaaatgaaaacaaaacaaccaaataattaatagtctctgcagaccaaagcgtaaatggattaacaaataacactgaatgcaaattcaggtaaccatatcaaaccaagaggaaagaatgtggttcatcttttggaggagttgtctaaaaggatccaatcaatcacaacctctctttttctctgcaatgatacaccagttaccatgatcattcccagaactcaggatacggagctctgacacattctccttgagcagactgcagagctccccttctcgaaacacatggtagtagcgcataaaggctgtggagtccaaaacatcagtctgtggatcttcgacagacattgtatcatctgggttgaaatctgtggaatcaactgcagaaatccttctcaatattttactagcagaaggattatcatcttctatgttgcctgcatccacacaattcacaccagtattagtgctatccagaaaatttccccctccatttctcctcatttccccttgatggtctccatttaaatgtttcagagtgcctggtgctctcagccactccaagtgttttccagaagaagattccacaaacacttcctcatctaaactttgcccttttgttgaaaatggctcttggtgatcaaagtctaaactagagtgtctggaaggctggactgttacagtgctactggcccaaacttctgtgtttttcaagggtcttactctttcaatttgcttcctcagagtcgattcatccaaagatctggagaaaaaccaggaacgaaacgattttcctaatgtgctgtaaaatccatattcttcctcgccttccttagaaatatttgcaaaacaggttcttgccatagcaggttcatagcccacgctgtgggaccgttttgaaccacactgctctttaaaacaaacagaacagctacactcagagcaaggaggatggtagggatggcctctttctgggtatccacactgcctcttcctcccagactggctggactctgagaagagctgggaacacagagccctgttccatggaacaagcacgtcttgcttctcaaagtgacggttcttttgttccattgcccaaacgtaaatcatcagttggcctccgggaactaagaccctggccatttcttttattgctctgattcttctttgttttgtagaaaaatgatgtatgactcctatggagatgatggcatcgaagccctcatccctaaaggggagattaaggttgtcacataccatggcttcacatcctctattccgggcaatctctaccagtggcccacagtagtcacagcccacggtatgtacctggctgttcactttaagatattttccagtcccacaacctatgtcagcgatgaggctgcctggcttctgctcttgcaggaactggcggacacgaggccaggctttgctctgcaggtcgctgaagtaaggggctgtgctctcgtacacattgtgcacatgctgcttctccagctgggcggcttcatgatccatcctgagtcatcctgtgattacaggaaaattacctcttgtctttgtgaatcacggcagtctccacctccagagagtgacagttgcttctcataactttctcaatgtgtaacgtaaatgaaaacttgtaggagtgaaatgaaatagtgcggtccttctcatgataaacctcttgtgtgagtctctgaaggaagcacaggccctggaagaaaaccaggtggtattggtgttatcaccaggtgaggggctaaagtttattcagcaacagtgaggtcaccaaggatctccaaaagttctgcctcgttatgcatggttggccttctgtttctgagttccacacggaccaatctgaccaaccaggcggccagacccgggcgcgggctccggggcacgcgctagacgacctgtcgcgccccctcctccctgcgggcgggcgccgaggcagcggatctagggcgcaacagaagcttctctccgctcccctatgcagaccattgtcagtgctccggtcgccggcgctttccgcacggtgtggcga

SEQ ID NO: 13887 - RNA, 2493 nt, Homo sapiens
  source 1..2493: mol_type = other RNA
gctgggattacaggcatgagccaccatgctcagcctaacagtgcctttaaaaacctcctgggctacattgaaaaccttattatcacatgtcaacttattttgaagcaagtttgcttataatttagtaaagtccttgtaaaacttcttgtttctctccactgtcactcagttttctgaaaactttaagtagaagcaaggccttggcaacaagataactcatcacatggttcaaagtatatctgtgcaatggatcaaatttacctattatcttgcacactgctctcagttataacctgagaaccagaaattatcccctcactttataaaaataccgttttaaaagattatttaacagcataatctttttaaatcaatgtgtaatactgaaaaacactatacatgtattttatctctctggggttaaaaaaaagtctgaggtgtactgaagggtactttctgttgcttcttcagatcttgtatattaacatttaagcacaaataccctttgtcaagtgctttcaatgccagaatctgtgcttattcaaaaatgaaaacaaaacaaccaaataattaatagtctctgcagaccaaagcgtaaatggattaacaaataacactgaatgcaaattcaggtaaccatatcaaaccaagaggaaagaatgtggttcatcttttggaggagttgtctaaaaggatccaatcaatcacaacctctctttttctctgcaatgatacaccagttaccatgatcattcccagaactcaggatacggagctctgacacattctccttgagcagactgcagagctccccttctcgaaacacatggtagtagcgcataaaggctgtggagtccaaaacatcagtctgtggatcttcgacagacattgtatcatctgggttgaaatctgtggaatcaactgcagaaatccttctcaatattttactagcagaaggattatcatcttctatgttgcctgcatccacacaattcacaccagtattagtgctatccagaaaatttccccctccatttctcctcatttccccttgatggtctccatttaaatgtttcagagtgcctggtgctctcagccactccaagtgttttccagaagaagattccacaaacacttcctcatctaaactttgcccttttgttgaaaatggctcttggtgatcaaagtctaaactagagtgtctggaaggctggactgttacagtgctactggcccaaacttctgtgtttttcaagggtcttactctttcaatttgcttcctcagagtcgattcatccaaagatctggagaaaaaccaggaacgaaacgattttcctaatgtgctgtaaaatccatattcttcctcgccttccttagaaatatttgcaaaacaggttcttgccatagcaggttcatagcccacgctgtgggaccgttttgaaccacactgctctttaaaacaaacagaacagctacactcagagcaaggaggatggtagggatggcctctttctgggtatccacactgcctcttcctcccagactggctggactctgagaagagctgggaacacagagccctgttccatggaacaagcacgtcttgcttctcaaagtgacggttcttttgttccattgcccaaacgtaaatcatcagttggcctccgggaactaagaccctggccatttcttttattgctctgattcttctttgttttgtagaaaaatgatgtatgactcctatggagatgatggcatcgaagccctcatccctaaaggggagattaaggttgtcacataccatggcttcacatcctctattccgggcaatctctaccagtggcccacagtagtcacagcccacggtatgtacctggctgttcactttaagatattttccagtcccacaacctatgtcagcgatgaggctgcctggcttctgctcttgcaggaactggcggacacgaggccaggctttgctctgcaggtcgctgaagtaaggggctgtgctctcgtacacattgtgcacatgctgcttctccagctgggcggcttcatgatccatcctgagtcatcctgtgattacaggaaaattacctcttgtctttgtgaatcacggcagtctccacctccagagagtgacagttgcttctcataactttctcaatgtgtaacgtaaatgaaaacttgtaggagtgaaatgaaatagtgcggtccttctcatgataaacctcttgtgtgagtctctgaaggaagcacaggccctggaagaaaaccaggtggtattggtgttatcaccaggtgaggggctaaagtttattcagcaacagtgaggtcaccaaggatctccaaaagttctgcctcgttatgcatggttggccttctgtttctgagttccacacggaccaatctgaccaactgtgtatcaaaaatatttaaaatcagaatcatgcctgtaattccagcattttgggaagctgaggtgggaggatg

SEQ ID NO: 13888 - RNA, 2604 nt, Homo sapiens
  source 1..2604: mol_type = other RNA
gctgggattacaggcatgagccaccatgctcagcctaacagtgcctttaaaaacctcctgggctacattgaaaaccttattatcacatgtcaacttattttgaagcaagtttgcttataatttagtaaagtccttgtaaaacttcttgtttctctccactgtcactcagttttctgaaaactttaagtagaagcaaggccttggcaacaagataactcatcacatggttcaaagtatatctgtgcaatggatcaaatttacctattatcttgcacactgctctcagttataacctgagaaccagaaattatcccctcactttataaaaataccgttttaaaagattatttaacagcataatctttttaaatcaatgtgtaatactgaaaaacactatacatgtattttatctctctggggttaaaaaaaagtctgaggtgtactgaagggtactttctgttgcttcttcagatcttgtatattaacatttaagcacaaataccctttgtcaagtgctttcaatgccagaatctgtgcttattcaaaaatgaaaacaaaacaaccaaataattaatagtctctgcagaccaaagcgtaaatggattaacaaataacactgaatgcaaattcaggtaaccatatcaaaccaagaggaaagaatgtggttcatcttttggaggagttgtctaaaaggatccaatcaatcacaacctctctttttctctgcaatgatacaccagttaccatgatcattcccagaactcaggatacggagctctgacacattctccttgagcagactgcagagctccccttctcgaaacacatggtagtagcgcataaaggctgtggagtccaaaacatcagtctgtggatcttcgacagacattgtatcatctgggttgaaatctgtggaatcaactgcagaaatccttctcaatattttactagcagaaggattatcatcttctatgttgcctgcatccacacaattcacaccagtattagtgctatccagaaaatttccccctccatttctcctcatttccccttgatggtctccatttaaatgtttcagagtgcctggtgctctcagccactccaagtgttttccagaagaagattccacaaacacttcctcatctaaactttgcccttttgttgaaaatggctcttggtgatcaaagtctaaactagagtgtctggaaggctggactgttacagtgctactggcccaaacttctgtgtttttcaagggtcttactctttcaatttgcttcctcagagtcgattcatccaaagatctggagaaaaaccaggaacgaaacgattttcctaatgtgctgtaaaatccatattcttcctcgccttccttagaaatatttgcaaaacaggttcttgccatagcaggttcatagcccacgctgtgggaccgttttgaaccacactgctctttaaaacaaacagaacagctacactcagagcaaggaggatggtagggatggcctctttctgggtatccacactgcctcttcctcccagactggctggactctgagaagagctgggaacacagagccctgttccatggaacaagcacgtcttgcttctcaaagtgacggttcttttgttccattgcccaaacgtaaatcatcagttggcctccgggaactaagaccctggccatttcttttattgctctgattcttctttgttttgtagaaaaatgatgtatgactcctatggagatgatggcatcgaagccctcatccctaaaggggagattaaggttgtcacataccatggcttcacatcctctattccgggcaatctctaccagtggcccacagtagtcacagcccacggtatgtacctggctgttcactttaagatattttccagtcccacaacctatgtcagcgatgaggctgcctggcttctgctcttgcaggaactggcggacacgaggccaggctttgctctgcaggtcgctgaagtaaggggctgtgctctcgtacacattgtgcacatgctgcttctccagctgggcggcttcatgatccatcctgagtcatcctgtgattacaggaaaattacctcttgtctttgtgaatcacggcagtctccacctccagagagtgacagttgcttctcataactttctcaatgtgtaacgtaaatgaaaacttgtaggagtgaaatgaaatagtgcggtccttctcatgataaacctcttgtgtgagtctctgaaggaagcacaggcccttcctattttggcattccttcttaaactgtattttcatcgtgagctttgaaaactttctggcttcaagttatcttagttctttgcctcttactaattaaaaatcagttccccagggaaagatacacgtgcactccatgaaaaaatacgaatccactttaacccttaaggcactagacatgtcctttatctctgaattctgatttatccaatctcacacccaaagcacatcccgcaatcccttactgcatggctgtctcgcctgttttgatcgtattgcaaggctgtttgcaaggtaaacagccaccccgggctactggaaaggcaggggacgagcagga

SEQ ID NO: 13889 - RNA, 2558 nt, Homo sapiens
  source 1..2558: mol_type = other RNA
gctgggattacaggcatgagccaccatgctcagcctaacagtgcctttaaaaacctcctgggctacattgaaaaccttattatcacatgtcaacttattttgaagcaagtttgcttataatttagtaaagtccttgtaaaacttcttgtttctctccactgtcactcagttttctgaaaactttaagtagaagcaaggccttggcaacaagataactcatcacatggttcaaagtatatctgtgcaatggatcaaatttacctattatcttgcacactgctctcagttataacctgagaaccagaaattatcccctcactttataaaaataccgttttaaaagattatttaacagcataatctttttaaatcaatgtgtaatactgaaaaacactatacatgtattttatctctctggggttaaaaaaaagtctgaggtgtactgaagggtactttctgttgcttcttcagatcttgtatattaacatttaagcacaaataccctttgtcaagtgctttcaatgccagaatctgtgcttattcaaaaatgaaaacaaaacaaccaaataattaatagtctctgcagaccaaagcgtaaatggattaacaaataacactgaatgcaaattcaggtaaccatatcaaaccaagaggaaagaatgtggttcatcttttggaggagttgtctaaaaggatccaatcaatcacaacctctctttttctctgcaatgatacaccagttaccatgatcattcccagaactcaggatacggagctctgacacattctccttgagcagactgcagagctccccttctcgaaacacatggtagtagcgcataaaggctgtggagtccaaaacatcagtctgtggatcttcgacagacattgtatcatctgggttgaaatctgtggaatcaactgcagaaatccttctcaatattttactagcagaaggattatcatcttctatgttgcctgcatccacacaattcacaccagtattagtgctatccagaaaatttccccctccatttctcctcatttccccttgatggtctccatttaaatgtttcagagtgcctggtgctctcagccactccaagtgttttccagaagaagattccacaaacacttcctcatctaaactttgcccttttgttgaaaatggctcttggtgatcaaagtctaaactagagtgtctggaaggctggactgttacagtgctactggcccaaacttctgtgtttttcaagggtcttactctttcaatttgcttcctcagagtcgattcatccaaagatctggagaaaaaccaggaacgaaacgattttcctaatgtgctgtaaaatccatattcttcctcgccttccttagaaatatttgcaaaacaggttcttgccatagcaggttcatagcccacgctgtgggaccgttttgaaccacactgctctttaaaacaaacagaacagctacactcagagcaaggaggatggtagggatggcctctttctgggtatccacactgcctcttcctcccagactggctggactctgagaagagctgggaacacagagccctgttccatggaacaagcacgtcttgcttctcaaagtgacggttcttttgttccattgcccaaacgtaaatcatcagttggcctccgggaactaagaccctggccatttcttttattgctctgattcttctttgttttgtagaaaaatgatgtatgactcctatggagatgatggcatcgaagccctcatccctaaaggggagattaaggttgtcacataccatggcttcacatcctctattccgggcaatctctaccagtggcccacagtagtcacagcccacggtatgtacctggctgttcactttaagatattttccagtcccacaacctatgtcagcgatgaggctgcctggcttctgctcttgcaggaactggcggacacgaggccaggctttgctctgcaggtcgctgaagtaaggggctgtgctctcgtacacattgtgcacatgctgcttctccagctgggcggcttcatgatccatcctgagtcatcctgtgattacaggaaaattacctcttgtctttgtgaatcacggcagtctccacctccagagagtgacagttgcttctcataactttctcaatgtgtaacgtaaatgaaaacttgtaggagtgaaatgaaatagtgcggtccttctcatgataaacctcttgtgtgagtctctgaaggaagcacaggcccttgaaggaagactgcagagttgctaggagagctcacaggtttcatcactttcccagagggaggactgtgtaggattcagccttagatcctgaaagtctagtccagagccctgcacatggaagtactgaataagttgaaggaacatatgcatcaagaaaaaaaattcaaaacaaactaacaaaaaacacaaaaaatgaaaaaagaataaaacaaagaaaaaaagccaaaagaacatgtgcatctacttctgacatatacatgtgtgatcttttctgtactacacaatactgaat

SEQ ID NO: 13890 - RNA, 2105 nt, Homo sapiens
  source 1..2105: mol_type = other RNA
gctgggattacaggcatgagccaccatgctcagcctaacagtgcctttaaaaacctcctgggctacattgaaaaccttattatcacatgtcaacttattttgaagcaagtttgcttataatttagtaaagtccttgtaaaacttcttgtttctctccactgtcactcagttttctgaaaactttaagtagaagcaaggccttggcaacaagataactcatcacatggttcaaagtatatctgtgcaatggatcaaatttacctattatcttgcacactgctctcagttataacctgagaaccagaaattatcccctcactttataaaaataccgttttaaaagattatttaacagcataatctttttaaatcaatgtgtaatactgaaaaacactatacatgtattttatctctctggggttaaaaaaaagtctgaggtgtactgaagggtactttctgttgcttcttcagatcttgtatattaacatttaagcacaaataccctttgtcaagtgctttcaatgccagaatctgtgcttattcaaaaatgaaaacaaaacaaccaaataattaatagtctctgcagaccaaagcgtaaatggattaacaaataacactgaatgcaaattcaggtaaccatatcaaaccaagaggaaagaatgtggttcatcttttggaggagttgtctaaaaggatccaatcaatcacaacctctctttttctctgcaatgatacaccagttaccatgatcattcccagaactcaggatacggagctctgacacattctccttgagcagactgcagagctccccttctcgaaacacatggtagtagcgcataaaggctgtggagtccaaaacatcagtctgtggatcttcgacagacattgtatcatctgggttgaaatctgtggaatcaactgcagaaatccttctcaatattttactagcagaaggattatcatcttctatgttgcctgcatccacacaattcacaccagtattagtgctatccagaaaatttccccctccatttctcctcatttccccttgatggtctccatttaaatgtttcagagtgcctggtgctctcagccactccaagtgttttccagaagaagattccacaaacacttcctcatctaaactttgcccttttgttgaaaatggctcttggtgatcaaagtctaaactagagtgtctggaaggctggactgttacagtgctactggcccaaacttctgtgtttttcaagggtcttactctttcaatttgcttcctcagagtcgattcatccaaagatctggagaaaaaccaggaacgaaacgattttcctaatgtgctgtaaaatccatattcttcctcgccttccttagaaatatttgcaaaacaggttcttgccatagcaggttcatagcccacgctgtgggaccgttttgaaccacactgctctttaaaacaaacagaacagctacactcagagcaaggaggatggtagggatggcctctttctgggtatccacactgcctcttcctcccagactggctggactctgagaagagctgggaacacagagccctgttccatggaacaagcacgtcttgcttctcaaagtgacggttcttttgttccattgcccaaacgtaaatcatcagttggcctccgggaactaagaccctggccatttcttttattgctctgattcttctttgttttgtagaaaaatgatgtatgactcctatggagatgatggcatcgaagccctcatccctaaaggggagattaaggttgtcacataccatggcttcacatcctctattccgggcaatctctaccagtggcccacagtagtcacagcccacggtatgtacctggctgttcactttaagatattttccagtcccacaacctatgtcagcgatgaggctgcctggttacctatgtcagcgatgaggctgcctggttacctatgtcagcgatgaggctgcctggttacctatgtcagcgatgaggctgcctggcttctgctcttgcaggaactggcggacacgaggccaggctttgctctgcaggtcgctgaagtaaggggctgtgctctcgtac

SEQ ID NO: 13891 - RNA, 2525 nt, Homo sapiens
  source 1..2525: mol_type = other RNA
gctgggattacaggcatgagccaccatgctcagcctaacagtgcctttaaaaacctcctgggctacattgaaaaccttattatcacatgtcaacttattttgaagcaagtttgcttataatttagtaaagtccttgtaaaacttcttgtttctctccactgtcactcagttttctgaaaactttaagtagaagcaaggccttggcaacaagataactcatcacatggttcaaagtatatctgtgcaatggatcaaatttacctattatcttgcacactgctctcagttataacctgagaaccagaaattatcccctcactttataaaaataccgttttaaaagattatttaacagcataatctttttaaatcaatgtgtaatactgaaaaacactatacatgtattttatctctctggggttaaaaaaaagtctgaggtgtactgaagggtactttctgttgcttcttcagatcttgtatattaacatttaagcacaaataccctttgtcaagtgctttcaatgccagaatctgtgcttattcaaaaatgaaaacaaaacaaccaaataattaatagtctctgcagaccaaagcgtaaatggattaacaaataacactgaatgcaaattcaggtaaccatatcaaaccaagaggaaagaatgtggttcatcttttggaggagttgtctaaaaggatccaatcaatcacaacctctctttttctctgcaatgatacaccagttaccatgatcattcccagaactcaggatacggagctctgacacattctccttgagcagactgcagagctccccttctcgaaacacatggtagtagcgcataaaggctgtggagtccaaaacatcagtctgtggatcttcgacagacattgtatcatctgggttgaaatctgtggaatcaactgcagaaatccttctcaatattttactagcagaaggattatcatcttctatgttgcctgcatccacacaattcacaccagtattagtgctatccagaaaatttccccctccatttctcctcatttccccttgatggtctccatttaaatgtttcagagtgcctggtgctctcagccactccaagtgttttccagaagaagattccacaaacacttcctcatctaaactttgcccttttgttgaaaatggctcttggtgatcaaagtctaaactagagtgtctggaaggctggactgttacagtgctactggcccaaacttctgtgtttttcaagggtcttactctttcaatttgcttcctcagagtcgattcatccaaagatctggagaaaaaccaggaacgaaacgattttcctaatgtgctgtaaaatccatattcttcctcgccttccttagaaatatttgcaaaacaggttcttgccatagcaggttcatagcccacgctgtgggaccgttttgaaccacactgctctttaaaacaaacagaacagctacactcagagcaaggaggatggtagggatggcctctttctgggtatccacactgcctcttcctcccagactggctggactctgagaagagctgggaacacagagccctgttccatggaacaagcacgtcttgcttctcaaagtgacggttcttttgttccattgcccaaacgtaaatcatcagttggcctccgggaactaagaccctggccatttcttttattgctctgattcttctttgttttgtagaaaaatgatgtatgactcctatggagatgatggcatcgaagccctcatccctaaaggggagattaaggttgtcacataccatggcttcacatcctctattccgggcaatctctaccagtggcccacagtagtcacagcccacggtatgtacctggctgttcactttaagatattttccagtcccacaacctgagtcatcctgtgattacaggaaaattacctcttgtctttgtgaatcacggcagtctccacctccagagagtgacagttgcttctcataactttctcaatgtgtaacgtaaatgaaaacttgtaggagtgaaatgaaatagtgcggtccttctcatgataaacctcttgtgtgagtctctgaaggaagcacaggccccaggcggccagacccgggcgcgggctccggggcacgcgctagacgacctgtcgcgccccctcctccctgcgggcgggcgccgaggcagcggatctagggcgcaacagaagcttctctccgctcccctatgcagaccattgtcagtgctccggtcgccggcgctttccgcacggtgtggcgactggcagcagctctcccgttgcgagtagtcacagcgctgtcccgcagccaggggcaaaagctgcttttgcatcagagccgagggctgcaccaggtgtaacttccaccccttgacctattttagagtgtgaggatgaaaggaagaggaaaaaatagacggagggcgcgcgggggtgcgggcggcagggtgcgcgcgtggccgtgggggagcgcgcgcgcgggccggggctcgtgt

SEQ ID NO: 13892 - RNA, 2765 nt, Homo sapiens
  source 1..2765: mol_type = other RNA
gctgggattacaggcatgagccaccatgctcagcctaacagtgcctttaaaaacctcctgggctacattgaaaaccttattatcacatgtcaacttattttgaagcaagtttgcttataatttagtaaagtccttgtaaaacttcttgtttctctccactgtcactcagttttctgaaaactttaagtagaagcaaggccttggcaacaagataactcatcacatggttcaaagtatatctgtgcaatggatcaaatttacctattatcttgcacactgctctcagttataacctgagaaccagaaattatcccctcactttataaaaataccgttttaaaagattatttaacagcataatctttttaaatcaatgtgtaatactgaaaaacactatacatgtattttatctctctggggttaaaaaaaagtctgaggtgtactgaagggtactttctgttgcttcttcagatcttgtatattaacatttaagcacaaataccctttgtcaagtgctttcaatgccagaatctgtgcttattcaaaaatgaaaacaaaacaaccaaataattaatagtctctgcagaccaaagcgtaaatggattaacaaataacactgaatgcaaattcaggtaaccatatcaaaccaagaggaaagaatgtggttcatcttttggaggagttgtctaaaaggatccaatcaatcacaacctctctttttctctgcaatgatacaccagttaccatgatcattcccagaactcaggatacggagctctgacacattctccttgagcagactgcagagctccccttctcgaaacacatggtagtagcgcataaaggctgtggagtccaaaacatcagtctgtggatcttcgacagacattgtatcatctgggttgaaatctgtggaatcaactgcagaaatccttctcaatattttactagcagaaggattatcatcttctatgttgcctgcatccacacaattcacaccagtattagtgctatccagaaaatttccccctccatttctcctcatttccccttgatggtctccatttaaatgtttcagagtgcctggtgctctcagccactccaagtgttttccagaagaagattccacaaacacttcctcatctaaactttgcccttttgttgaaaatggctcttggtgatcaaagtctaaactagagtgtctggaaggctggactgttacagtgctactggcccaaacttctgtgtttttcaagggtcttactctttcaatttgcttcctcagagtcgattcatccaaagatctggagaaaaaccaggaacgaaacgattttcctaatgtgctgtaaaatccatattcttcctcgccttccttagaaatatttgcaaaacaggttcttgccatagcaggttcatagcccacgctgtgggaccgttttgaaccacactgctctttaaaacaaacagaacagctacactcagagcaaggaggatggtagggatggcctctttctgggtatccacactgcctcttcctcccagactggctggactctgagaagagctgggaacacagagccctgttccatggaacaagcacgtcttgcttctcaaagtgacggttcttttgttccattgcccaaacgtaaatcatcagttggcctccgggaactaagaccctggccatttcttttattgctctgattcttctttgttttgtagaaaaatgatgtatgactcctatggagatgatggcatcgaagccctcatccctaaaggggagattaaggttgtcacataccatggcttcacatcctctattccgggcaatctctaccagtggcccacagtagtcacagcccacggtatgtacctggctgttcactttaagatattttccagtcccacaacttgctgctgacttgactgtctcgagtttctgctgtaaaatgaatattctaggtactggcatgccaagggtgcaatttcaggattcctatgtcagcgatgaggctgcctggcttctgctcttgcaggaactggcggacacgaggccaggctttgctctgcaggtcgctgaagtaaggggctgtgctctcgtacacattgtgcacatgctgcttctccagctgggcggcttcatgatccatcctgagtcatcctgtgattacaggaaaattacctcttgtctttgtgaatcacggcagtctccacctccagagagtgacagttgcttctcataactttctcaatgtgtaacgtaaatgaaaacttgtaggagtgaaatgaaatagtgcggtccttctcatgataaacctcttgtgtgagtctctgaaggaagcacaggccccaggcggccagacccgggcgcgggctccggggcacgcgctagacgacctgtcgcgccccctcctccctgcgggcgggcgccgaggcagcggatctagggcgcaacagaagcttctctccgctcccctatgcagaccattgtcagtgctccggtcgccggcgctttccgcacggtgtggcgactggcagcagctctcccgttgcgagtagtcacagcgctgtcccgcagccaggggcaaaagctgcttttgcatcagagccgagggctgcaccaggtgtaacttccaccccttgacctattttagagtgtgaggatgaaaggaagaggaaaaaatagacggagggcgcgcgggggtgcgggcggcagggtgcgcgcgtggccgtgggggagcgcgcgcgcgggccggggctcgtgt

SEQ ID NO: 13893 - RNA, 2698 nt, Homo sapiens
  source 1..2698: mol_type = other RNA
gctgggattacaggcatgagccaccatgctcagcctaacagtgcctttaaaaacctcctgggctacattgaaaaccttattatcacatgtcaacttattttgaagcaagtttgcttataatttagtaaagtccttgtaaaacttcttgtttctctccactgtcactcagttttctgaaaactttaagtagaagcaaggccttggcaacaagataactcatcacatggttcaaagtatatctgtgcaatggatcaaatttacctattatcttgcacactgctctcagttataacctgagaaccagaaattatcccctcactttataaaaataccgttttaaaagattatttaacagcataatctttttaaatcaatgtgtaatactgaaaaacactatacatgtattttatctctctggggttaaaaaaaagtctgaggtgtactgaagggtactttctgttgcttcttcagatcttgtatattaacatttaagcacaaataccctttgtcaagtgctttcaatgccagaatctgtgcttattcaaaaatgaaaacaaaacaaccaaataattaatagtctctgcagaccaaagcgtaaatggattaacaaataacactgaatgcaaattcaggtaaccatatcaaaccaagaggaaagaatgtggttcatcttttggaggagttgtctaaaaggatccaatcaatcacaacctctctttttctctgcaatgatacaccagttaccatgatcattcccagaactcaggatacggagctctgacacattctccttgagcagactgcagagctccccttctcgaaacacatggtagtagcgcataaaggctgtggagtccaaaacatcagtctgtggatcttcgacagacattgtatcatctgggttgaaatctgtggaatcaactgcagaaatccttctcaatattttactagcagaaggattatcatcttctatgttgcctgcatccacacaattcacaccagtattagtgctatccagaaaatttccccctccatttctcctcatttccccttgatggtctccatttaaatgtttcagagtgcctggtgctctcagccactccaagtgttttccagaagaagattccacaaacacttcctcatctaaactttgcccttttgttgaaaatggctcttggtgatcaaagtctaaactagagtgtctggaaggctggactgttacagtgctactggcccaaacttctgtgtttttcaagggtcttactctttcaatttgcttcctcagagtcgattcatccaaagatctggagaaaaaccaggaacgaaacgattttcctaatgtgctgtaaaatccatattcttcctcgccttccttagaaatatttgcaaaacaggttcttgccatagcaggttcatagcccacgctgtgggaccgttttgaaccacactgctctttaaaacaaacagaacagctacactcagagcaaggaggatggtagggatggcctctttctgggtatccacactgcctcttcctcccagactggctggactctgagaagagctgggaacacagagccctgttccatggaacaagcacgtcttgcttctcaaagtgacggttcttttgttccattgcccaaacgtaaatcatcagttggcctccgggaactaagaccctggccatttcttttattgctctgattcttctttgttttgtagaaaaatgatgtatgactcctatggagatgatggcatcgaagccctcatccctaaaggggagattaaggttgtcacataccatggcttcacatcctctattccgggcaatctctaccagtggcccacagtagtcacagcccacggtatgtacctggctgttcactttaagatattttccagtcccacaacttgctgctgacttgactgtctcgagtttctgctgtaaaatgaatattctaggtactggcatgccaagggtgcaatttcaggattcctatgtcagcgatgaggctgcctggcttctgctcttgcaggaactggcggacacgaggccaggctttgctctgcaggtcgctgaagtaaggggctgtgctctcgtacacattgtgcacatgctgcttctccagctgggcggcttcatgatccatcctgagtcatcctgtgattacaggaaaattacctcttgtctttgtgaatcacggcagtctccacctccagagagtgacagttgcttctcataactttctcaatgtgtaacgtaaatgaaaacttgtaggagtgaaatgaaatagtgcggtccttctcatgataaacctcttgtgtgagtctctgaaggaagcacaggccccaggcggccagacccgggcgcgggctccggggcacgcgctagacgacctgtcgcgccccctcctccctgcgggcgggcgccgaggcagcggatctagggcgcaacagaagcttctctccgctcccctatgcagaccattgtcagtgctccggtcgccggcgctttccgcacggtgtggcgactggcagcagctctcccgttgcgagtagtcacagcgctgtcccgcagccaggggcaaaagctgcttttgcatcagagccgagggctgcaccaggtgtaacttccaccccttgaccttgggtgacgacgacgcttggctttagcgcggctcttctcacttaatttttt

SEQ ID NO: 13894 - RNA, 2727 nt, Homo sapiens
  source 1..2727: mol_type = other RNA
gctgggattacaggcatgagccaccatgctcagcctaacagtgcctttaaaaacctcctgggctacattgaaaaccttattatcacatgtcaacttattttgaagcaagtttgcttataatttagtaaagtccttgtaaaacttcttgtttctctccactgtcactcagttttctgaaaactttaagtagaagcaaggccttggcaacaagataactcatcacatggttcaaagtatatctgtgcaatggatcaaatttacctattatcttgcacactgctctcagttataacctgagaaccagaaattatcccctcactttataaaaataccgttttaaaagattatttaacagcataatctttttaaatcaatgtgtaatactgaaaaacactatacatgtattttatctctctggggttaaaaaaaagtctgaggtgtactgaagggtactttctgttgcttcttcagatcttgtatattaacatttaagcacaaataccctttgtcaagtgctttcaatgccagaatctgtgcttattcaaaaatgaaaacaaaacaaccaaataattaatagtctctgcagaccaaagcgtaaatggattaacaaataacactgaatgcaaattcaggtaaccatatcaaaccaagaggaaagaatgtggttcatcttttggaggagttgtctaaaaggatccaatcaatcacaacctctctttttctctgcaatgatacaccagttaccatgatcattcccagaactcaggatacggagctctgacacattctccttgagcagactgcagagctccccttctcgaaacacatggtagtagcgcataaaggctgtggagtccaaaacatcagtctgtggatcttcgacagacattgtatcatctgggttgaaatctgtggaatcaactgcagaaatccttctcaatattttactagcagaaggattatcatcttctatgttgcctgcatccacacaattcacaccagtattagtgctatccagaaaatttccccctccatttctcctcatttccccttgatggtctccatttaaatgtttcagagtgcctggtgctctcagccactccaagtgttttccagaagaagattccacaaacacttcctcatctaaactttgcccttttgttgaaaatggctcttggtgatcaaagtctaaactagagtgtctggaaggctggactgttacagtgctactggcccaaacttctgtgtttttcaagggtcttactctttcaatttgcttcctcagagtcgattcatccaaagatctggagaaaaaccaggaacgaaacgattttcctaatgtgctgtaaaatccatattcttcctcgccttccttagaaatatttgcaaaacaggttcttgccatagcaggttcatagcccacgctgtgggaccgttttgaaccacactgctctttaaaacaaacagaacagctacactcagagcaaggaggatggtagggatggcctctttctgggtatccacactgcctcttcctcccagactggctggactctgagaagagctgggaacacagagccctgttccatggaacaagcacgtcttgcttctcaaagtgacggttcttttgttccattgcccaaacgtaaatcatcagttggcctccgggaactaagaccctggccatttcttttattgctctgattcttctttgttttgtagaaaaatgatgtatgactcctatggagatgatggcatcgaagccctcatccctaaaggggagattaaggttgtcacataccatggcttcacatcctctattccgggcaatctctaccagtggcccacagtagtcacagcccacggtatgtacctggctgttcactttaagatattttccagtcccacaacttgctgctgacttgactgtctcgagtttctgctgtaaaatgaatattctaggtactggcatgccaagggtgcaatttcaggattcctatgtcagcgatgaggctgcctggttacctatgtcagcgatgaggctgcctggttacctatgtcagcgatgaggctgcctggttacctatgtcagcgatgaggctgcctggcttctgctcttgcaggaactggcggacacgaggccaggctttgctctgcaggtcgctgaagtaaggggctgtgctctcgtacacattgtgcacatgctgcttctccagctgggcggcttcatgatccatcctcttgtctttgtgaatcacggcagtctccacctccagagagtgacagttgcttctcataactttctcaatgtgtaacgtaaatgaaaacttgtaggagtgaaatgaaatagtgcggtccttctcatgataaacctcttgtgtgagtctctgaaggaagcacaggccccaggcggccagacccgggcgcgggctccggggcacgcgctagacgacctgtcgcgccccctcctccctgcgggcgggcgccgaggcagcggatctagggcgcaacagaagcttctctccgctcccctatgcagaccattgtcagtgctccggtcgccggcgctttccgcacggtgtggcgactggcagcagctctcccgttgcgagtagtcacagcgctgtcccgcagccaggggcaaaagctgcttttgcatcagagccgagggctgcaccaggtgtaacttccaccccttgaccttgggtgacgacgacgcttggcttt

SEQ ID NO: 13895 - RNA, 2985 nt, Homo sapiens
  source 1..2985: mol_type = other RNA
gctgggattacaggcatgagccaccatgctcggccatgagttggaactcttgatcaggcccctctgagttcaccatgccatgctcaggctgctttcatcaacagagccaaagcacttgacctcttcgtgccttggttttgccatccatgaaacaggaaaataatcctagcgtcagaaatataaaatgttgtccttgcctggcagcctttggaagatccacctctttgggatggcagtagggaggtgtgctctcctggcagcacgggctgcctgcggcccttgctggacaggagaattctggaaaacaacttcattcctgtcttcagtagatctgacaggcccagaggagaaagcctgcactcttccctgtgtctgtggcactcctccaggtgtctgcatggccctctccatagtgacctatgtgtaaatgtcatcgcttctaaaagagccactctgcccagctcagctccaccactttctcttcttaccctgcttttttctcttttttagttctggaagctgaaagtacaacaggaaggtgttggcagggttggttccttctgacagctgtaaggcagggtctgttccacgcctctcccctggcttctggtggtttgctggtcctcttaggtgttccttggcttgcagatgcattatcccgacctcagccttcacgtggcgttctccccatgtgcgtttctctctgcgtcccacttcctccttcattgttttgtgatggagccagcagccgcgcagtgtgatccaaagacgcctggtggagggaaacccgaattggcttcagggggagcctccccggatgcaggacctgattcatggccaggagagcaggaggaagaccagcaggacagagattccagctcttctggtcaactgcaaggtgagaggcctcccagggacacactttcattaacaaccctgcctgcactcacttcacctgctctcctttctgctctgccctgatgggagagggagggagggagaaagggcacctctctccctagcctggacctaaccaggatcctctacctccttcctccctgccccaagccatgtctcctcggtgcaactccatctgtcaccaccattactctgccccccttccttggtcaaaatacaatacttaaattaagtaagtactcctcagtgtgctctacacagacaaatggtgtgtgtgcatggataacgtaattctggaaaaaactcatgtgttctaaggcattggccctgtaatctctggaaccacttaaccactcagtcactattgaacattcgcaataaattcccactggtcctcggccaccgtctttgctctgtgcttcttctatgtggattgctcttcttgctctccaatcattctgggtccgcattctttagggggtagggtgggggttcagaagaatccttcaccagctatgaggcaagtacagctaggtgggatcctggaggcttgagggagcacactgtggtggctggtctggatggtagagcgtttggtgaagcagggcacgagtcacagggaggtcgtcaggatccacgcccagctcctgcagcaggctgtggtactccggcttggtctccagcagtttcaccagattggtagactccatccgctccagctgcacctcccagtacacatagatcttctggttgaaagtgacatatacgaggcaggggctgttgcggccctctttgcaggcgtacaggcctgcacagaaggcacggatattttcatccacttggaagcggacgacggtgcggttgtgatcaatgatatatgtctgtccatcccaggcgcatgcaactacctcctcatgcccgttgccggtgacatccagtttctccagggcaaagagctggtgatccacctgcactgaccacagcagcttgtctgcttcttccatttcttccatgagcttcagtgtcccatccagggtgcacagggcaaagaggccagagccactactctcagtgccgtggccttgtttgatgttgccaattaggtgagtggagacattcttgttgtggatacggccagatgtctggtgcagcaccacgtctcgggcagctggggtctccctactaccatccgtgggcccttcagaggcaggaggggacccagtgtcctttttccaggtacacagtagaattgcatacgcacaacctggctgagacaccatcagttcaggaagacccagtggccccagagtcactgagaggctgtccacctgaccctccagcatccatttcttgagggacaccagctgccctgtcagatgttcaggaccctcacctagctcctcccagcggaaagctcgcaccacacggtctgtgtagcccaccaccagctcacgacacccatctccatcccaatcccttgggatatgctctagtatccactgactcctactctcctggctgcctgcaaaggtaggcatgcccaccgatgtcgctgatcagcatgaccttggtgttggcagggatgtgctgcttgaagactggacgctgctcctctccgattagtgtctcgtggtgcccagaagcatccaacaccttggcaggtgtcaggtcaaacaaatgaaaccagccttcagcactcactgccaccaacaggttctttcctttattacacacgtctccaaccccaacgcaagtcagcattccctggcaggaacaggtgagccatggccgactgtcatcatttttatacacagacaccttcccgctggtgtctcccaccaccagttcatttaacgtatcgttatcaacgtctccgaggcagattgcgtgcgggaagaggctcccgctgaactccagcgccacgcgctgcacgtagctaactgacctcatggcacctccaagagcagagggagcggagaggcccagtaaatattccctgaacccccgtcgcgacagccgccagagcggaaggccacctaaggcagcaagttacgtcactgcctgaac

SEQ ID NO: 13896 - RNA, 2890 nt, Homo sapiens
  source 1..2890: mol_type = other RNA
gctgggattacaggcatgagccaccatgctcggccatgagttggaactcttgatcaggcccctctgagttcaccatgccatgctcaggctgctttcatcaacagagccaaagcacttgacctcttcgtgccttggttttgccatccatgaaacaggaaaataatcctagcgtcagaaatataaaatgttgtccttgcctggcagcctttggaagatccacctctttgggatggcagtagggaggtgtgctctcctggcagcacgggctgcctgcggcccttgctggacaggagaattctggaaaacaacttcattcctgtcttcagtagatctgacaggcccagaggagaaagcctgcactcttccctgtgtctgtggcactcctccaggtgtctgcatggccctctccatagtgacctatgtgtaaatgtcatcgcttctaaaagagccactctgcccagctcagctccaccactttctcttcttaccctgcttttttctcttttttagttctggaagctgaaagtacaacaggaaggtgttggcagggttggttccttctgacagctgtaaggcagggtctgttccacgcctctcccctggcttctggtggtttgctggtcctcttaggtgttccttggcttgcagatgcattatcccgacctcagccttcacgtggcgttctccccatgtgcgtttctctctgcgtcccacttcctccttcattgttttgtgatggagccagcagccgcgcagtgtgatccaaagacgcctggtggagggaaacccgaattggcttcagggggagcctccccggatgcaggacctgattcatggccaggagagcaggaggaagaccagcaggacagagattccagctcttctggtcaactgcaaggtgagaggcctcccagggacacactttcattaacaaccctgcctgcactcacttcacctgctctcctttctgctctgccctgatgggagagggagggagggagaaagggcacctctctccctagcctggacctaaccaggatcctctacctccttcctccctgccccaagccatgtctcctcggtgcaactccatctgtcaccaccattactctgccccccttccttggtcaaaatacaatacttaaattaagtaagtactcctcagtgtgctctacacagacaaatggtgtgtgtgcatggataacgtaattctggaaaaaactcatgtgttctaaggcattggccctgtaatctctggaaccacttaaccactcagtcactattgaacattcgcaataaattcccactggtcctcggccaccgtctttgctctgtgcttcttctatgtggattgctcttcttgctctccaatcattctgggtccgcattctttagggggtagggtgggggttcagaagaatccttcaccagctatgaggcaagtacagctaggtgggatcctggaggcttgagggagcacactgtggtggctggtctggatggtagagcgtttggtgaagcagggcacgagtcacagggaggtcgtcaggatccacgcccagctcctgcagcaggctgtggtactccggcttggtctccagcagtttcaccagattggtagactccatccgctccagctgcacctcccagtacacatagatcttctggttgaaagtgacatatacgaggcaggggctgttgcggccctctttgcaggcgtacaggcctgcacagaaggcacggatattttcatccacttggaagcggacgacggtgcggttgtgatcaatgatatatgtctgtccatcccaggcgcatgcaactacctcctcatgcccgttgccggtgacatccagtttctccagggcaaagagctggtgatccacctgcactgaccacagcagcttgtctgcttcttccatttcttccatgagcttcagtgtcccatccagggtgcacagggcaaagaggccagagccactactctcagtgccgtggccttgtttgatgttgccaattaggtgagtggagacattcttgttgtggatacggccagatgtctggtgcagcaccacgtctcgggcagctggggtctccctactaccatccgtgggcccttcagaggcaggaggggacccagtgtcctttttccaggtacacagtagaattgcatacgcacaacctggctgagacaccatcagttcaggaagacccagtggccccagagtcactgagaggctgtccacctgaccctccagcatccatttcttgagggacaccagctgccctgtcagatgttcaggaccctcacctagctcctcccagcggaaagctcgcaccacacggtctgtgtagcccaccaccagctcacgacacccatctccatcgatgtcgctgatcagcatgaccttggtgttggcagggatgtgctgcttgaagactggacgctgctcctctccgattagtgtctcgtggtgcccagaagcatccaacaccttggcaggtgtcaggtcaaacaaatgaaaccagccttcagcactcactgccaccaacaggttctttcctttattacacacgtctccaaccccaacgcaagtcagcattccctggcaggaacaggtgagccatggccgactgtcatcatttttatacacagacaccttcccgctggtgtctcccaccaccagttcatttaacgtatcgttatcaacgtctccgaggcagattgcgtgcgggaagaggctcccgctgaactccagcgccacgcgctgcacgtagctaactgacctcatggcacctccaagagcagagggagcggagaggcccagtaaatattccctgaacccccgtcgcgacagccgccagagcggaaggccacctaaggcagcaa

SEQ ID NO: 13897 - RNA, 2960 nt, Homo sapiens
  source 1..2960: mol_type = other RNA
gctgggattacaggcatgagccaccatgctcggccatgagttggaactcttgatcaggcccctctgagttcaccatgccatgctcaggctgctttcatcaacagagccaaagcacttgacctcttcgtgccttggttttgccatccatgaaacaggaaaataatcctagcgtcagaaatataaaatgttgtccttgcctggcagcctttggaagatccacctctttgggatggcagtagggaggtgtgctctcctggcagcacgggctgcctgcggcccttgctggacaggagaattctggaaaacaacttcattcctgtcttcagtagatctgacaggcccagaggagaaagcctgcactcttccctgtgtctgtggcactcctccaggtgtctgcatggccctctccatagtgacctatgtgtaaatgtcatcgcttctaaaagagccactctgcccagctcagctccaccactttctcttcttaccctgcttttttctcttttttagttctggaagctgaaagtacaacaggaaggtgttggcagggttggttccttctgacagctgtaaggcagggtctgttccacgcctctcccctggcttctggtggtttgctggtcctcttaggtgttccttggcttgcagatgcattatcccgacctcagccttcacgtggcgttctccccatgtgcgtttctctctgcgtcccacttcctccttcattgttttgtgatggagccagcagccgcgcagtgtgatccaaagacgcctggtggagggaaacccgaattggcttcagggggagcctccccggatgcaggacctgattcatggccaggagagcaggaggaagaccagcaggacagagattccagctcttctggtcaactgcaaggtgagaggcctcccagggacacactttcattaacaaccctgcctgcactcacttcacctgctctcctttctgctctgccctgatgggagagggagggagggagaaagggcacctctctccctagcctggacctaaccaggatcctctacctccttcctccctgccccaagccatgtctcctcggtgcaactccatctgtcaccaccattactctgccccccttccttggtcaaaatacaatacttaaattaagtaagtactcctcagtgtgctctacacagacaaatggtgtgtgtgcatggataacgtaattctggaaaaaactcatgtgttctaaggcattggccctgtaatctctggaaccacttaaccactcagtcactattgaacattcgcaataaattcccactggtcctcggccaccgtctttgctctgtgcttcttctatgtggattgctcttcttgctctccaatcattctgggtccgcattctttagggggtagggtgggggttcagaagaatccttcaccagctatgaggcaagtacagctaggtgggatcctggaggcttgagggagcacactgtggtggctggtctggatggtagagcgtttggtgaagcagggcacgagtcacagggaggtcgtcaggatccacgcccagctcctgcagcatgctgtgggtctcctgggcactcgggccactggcttttctgggactcacccacgcccagctcctgcagcaggctgtggtactccggcttggtctccagcagtttcaccagattggtagactccatccgctccagctgcacctcccagtacacatagatcttctggttgaaagtgacatatacgaggcaggggctgttgcggccctctttgcaggcgtacaggcctgcacagaaggcacggatattttcatccacttggaagcggacgacggtgcggttgtgatcaatgatatatgtctgtccatcccaggcgcatgcaactacctcctcatgcccgttgccggtgacatccagtttctccagggcaaagagctggtgatccacctgcactgaccacagcagcttgtctgcttcttccatttcttccatgagcttcagtgtcccatccagggtgcacagggcaaagaggccagagccactactctcagtgccgtggccttgtttgatgttgccaattaggtgagtggagacattcttgttgtggatacggccagatgtctggtgcagcaccacgtctcgggcagctggggtctccctactaccatccgtgggcccttcagaggcaggaggggacccagtgtcctttttccaggtacacagtagaattgcatacgcacaacctggctgagacaccatcagttcaggaagacccagtggccccagagtcactgagaggctgtccacctgaccctccagcatccatttcttgagggacaccagctgccctgtcagatgttcaggaccctcacctagctcctcccagcggaaagctcgcaccacacggtctgtgtagcccaccaccagctcacgacacccatctccatcgatgtcgctgatcagcatgaccttggtgttggcagggatgtgctgcttgaagactggacgctgctcctctccgattagtgtctcgtggtgcccagaagcatccaacaccttggcaggtgtcaggtcaaacaaatgaaaccagccttcagcactcactgccaccaacaggttctttcctttattacacacgtctccaaccccaacgcaagtcagcattccctggcaggaacaggtgagccatggccgactgtcatcatttttatacacagacaccttcccgctggtgtctcccaccaccagttcatttaacgtatcgttatcaacgtctccgaggcagattgcgtgcgggaagaggctcccgctgaactccagcgccacgcgctgcacgtagctaactgacctcatggcacctccaagagcagagggagcggagaggcccagtaaatattccctgaacccccgtcgcgacagccgccagagcggaaggccacctaaggcagcaa

SEQ ID NO: 13898 - RNA, 2997 nt, Homo sapiens
  source 1..2997: mol_type = other RNA
gctgggattacaggcatgagccaccatgctcggccatgagttggaactcttgatcaggcccctctgagttcaccatgccatgctcaggctgctttcatcaacagagccaaagcacttgacctcttcgtgccttggttttgccatccatgaaacaggaaaataatcctagcgtcagaaatataaaatgttgtccttgcctggcagcctttggaagatccacctctttgggatggcagtagggaggtgtgctctcctggcagcacgggctgcctgcggcccttgctggacaggagaattctggaaaacaacttcattcctgtcttcagtagatctgacaggcccagaggagaaagcctgcactcttccctgtgtctgtggcactcctccaggtgtctgcatggccctctccatagtgacctatgtgtaaatgtcatcgcttctaaaagagccactctgcccagctcagctccaccactttctcttcttaccctgcttttttctcttttttagttctggaagctgaaagtacaacaggaaggtgttggcagggttggttccttctgacagctgtaaggcagggtctgttccacgcctctcccctggcttctggtggtttgctggtcctcttaggtgttccttggcttgcagatgcattatcccgacctcagccttcacgtggcgttctccccatgtgcgtttctctctgcgtcccacttcctccttcattgttttgtgatggagccagcagccgcgcagtgtgatccaaagacgcctggtggagggaaacccgaattggcttcagggggagcctccccggatgcaggacctgattcatggccaggagagcaggaggaagaccagcaggacagagattccagctcttctggtcaactgcaaggtgagaggcctcccagggacacactttcattaacaaccctgcctgcactcacttcacctgctctcctttctgctctgccctgatgggagagggagggagggagaaagggcacctctctccctagcctggacctaaccaggatcctctacctccttcctccctgccccaagccatgtctcctcggtgcaactccatctgtcaccaccattactctgccccccttccttggtcaaaatacaatacttaaattaagtaagtactcctcagtgtgctctacacagacaaatggtgtgtgtgcatggataacgtaattctggaaaaaactcatgtgttctaaggcattggccctgtaatctctggaaccacttaaccactcagtcactattgaacattcgcaataaattcccactggtcctcggccaccgtctttgctctgtgcttcttctatgtggattgctcttcttgctctccaatcattctgggtccgcattctttctctttggggtggggcaaaggctgagactttcactccctgcagcacgaggagttcccagagatgttctgactatcccccatctctgtgccagtgtcctcggatctttagggggtagggtgggggttcagaagaatccttcaccagctatgaggcaagtacagctaggtgggatcctggaggcttgagggagcacactgtggtggctggtctggatggtagagcgtttggtgaagcagggcacgagtcacagggaggtcgtcaggatccacgcccagctcctgcagcaggctgtggtactccggcttggtctccagcagtttcaccagattggtagactccatccgctccagctgcacctcccagtacacatagatcttctggttgaaagtgacatatacgaggcaggggctgttgcggccctctttgcaggcgtacaggcctgcacagaaggcacggatattttcatccacttggaagcggacgacggtgcggttgtgatcaatgatatatgtctgtccatcccaggcgcatgcaactacctcctcatgcccgttgccggtgacatccagtttctccagggcaaagagctggtgatccacctgcactgaccacagcagcttgtctgcttcttccatttcttccatgagcttcagtgtcccatccagggtgcacagggcaaagaggccagagccactactctcagtgccgtggccttgtttgatgttgccaattaggtgagtggagacattcttgttgtggatacggccagatgtctggtgcagcaccacgtctcgggcagctggggtctccctactaccatccgtgggcccttcagaggcaggaggggacccagtgtcctttttccaggtacacagtagaattgcatacgcacaacctggctgagacaccatcagttcaggaagacccagtggccccagagtcactgagaggctgtccacctgaccctccagcatccatttcttgagggacaccagctgccctgtcagatgttcaggaccctcacctagctcctcccagcggaaagctcgcaccacacggtctgtgtagcccaccaccagctcacgacacccatctccatcgatgtcgctgatcagcatgaccttggtgttggcagggatgtgctgcttgaagactggacgctgctcctctccgattagtgtctcgtggtgcccagaagcatccaacaccttggcaggtgtcaggtcaaacaaatgaaaccagccttcagcactcactgccaccaacaggttctttcctttattacacacgtctccaaccccaacgcaagtcagcattccctggcaggaacaggtgagccatggccgactgtcatcatttttatacacagacaccttcccgctggtgtctcccaccaccagttcatttaacgtatcgttatcaacgtctccgaggcagattgcgtgcgggaagaggctcccgctgaactccagcgccacgcgctgcacgtagctaactgacctcatggcacctccaagagcagagggagcggagaggcccagtaaatattccctgaacccccgtcgcgacagccgccagagcggaaggccacctaaggcagcaa

SEQ ID NO: 13899 - RNA, 2273 nt, Homo sapiens
  source 1..2273: mol_type = other RNA
gctgggattacaggcatgagccaccatgctcggccatgagttggaactcttgatcaggcccctctgagttcaccatgccatgctcaggctgctttcatcaacagagccaaagcacttgacctcttcgtgccttggttttgccatccatgaaacaggaaaataatcctagcgtcagaaatataaaatgttgtccttgcctggcagcctttggaagatccacctctttgggatggcagtagggaggtgtgctctcctggcagcacgggctgcctgcggcccttgctggacaggagaattctggaaaacaacttcattcctgtcttcagtagatctgacaggcccagaggagaaagcctgcactcttccctgtgtctgtggcactcctccaggtgtctgcatggccctctccatagtgacctatgtgtaaatgtcatcgcttctaaaagagccactctgcccagctcagctccaccactttctcttcttaccctgcttttttctcttttttagttctggaagctgaaagtacaacaggaaggtgttggcagggttggttccttctgacagctgtaaggcagggtctgttccacgcctctcccctggcttctggtggtttgctggtcctcttaggtgttccttggcttgcagatgcattatcccgacctcagccttcacgtggcgttctccccatgtgcgtttctctctgcgtcccacttcctccttcattgttttgtgatggagccagcagccgcgcagtgtgatccaaagacgcctttagggggtagggtgggggttcagaagaatccttcaccagctatgaggcaagtacagctaggtgggatcctggaggcttgagggagcacactgtggtggctggtctggatggtagagcgtttggtgaagcagggcacgagtcacagggaggtcgtcaggatccacgcccagctcctgcagcaggctgtggtactccggcttggtctccagcagtttcaccagattggtagactccatccgctccagctgcacctcccagtacacatagatcttctggttgaaagtgacatatacgaggcaggggctgttgcggccctctttgcaggcgtacaggcctgcacagaaggcacggatattttcatccacttggaagcggacgacggtgcggttgtgatcaatgatatatgtctgtccatcccaggcgcatgcaactacctcctcatgcccgttgccggtgacatccagtttctccagggcaaagagctggtgatccacctgcactgaccacagcagcttgtctgcttcttccatttcttccatgagcttcagtgtcccatccagggtgcacagggcaaagaggccagagccactactctcagtgccgtggccttgtttgatgttgccaattaggtgagtggagacattcttgttgtggatacggccagatgtctggtgcagcaccacgtctcgggcagctggggtctccctactaccatccgtgggcccttcagaggcaggaggggacccagtgtcctttttccaggtacacagtagaattgcatacgcacaacctggctgagacaccatcagttcaggaagacccagtggccccagagtcactgagaggctgtccacctgaccctccagcatccatttcttgagggacaccagctgccctgtcagatgttcaggaccctcacctagctcctcccagcggaaagctcgcaccacacggtctgtgtagcccaccaccagctcacgacacccatctccatcgatgtcgctgatcagcatgaccttggtgttggcagggatgtgctgcttgaagactggacgctgctcctctccgattagtgtctcgtggtgcccagaagcatccaacaccttggcaggtgtcaggtcaaacaaatgaaaccagccttcagcactcactgccaccaacaggttctttcctttattacacacgtctccaaccccaacgcaagtcagcattccctggcaggaacaggtgagccatggccgactgtcatcatttttatacacagacaccttcccgctggtgtctcccaccaccagttcatttaacgtatcgttatcaacgtctccgaggcagattgcgtgcgggaagaggctcccgctgaactccagcgccacgcgctgcacgtagctaactgacctcatggcacctccaagagcagagggagcggagaggcccagtaaatattccctgaacccccgtcgcgacagccgccagagcggaaggccacctaaggcagcaa

SEQ ID NO: 13900 - RNA, 2221 nt, Homo sapiens
  source 1..2221: mol_type = other RNA
gctgggattacaggcatgagccaccatgctcggccatgagttggaactcttgatcaggcccctctgagttcaccatgccatgctcaggctgctttcatcaacagagccaaagcacttgacctcttcgtgccttggttttgccatccatgaaacaggaaaataatcctagcgtcagaaatataaaatgttgtccttgcctggcagcctttggaagatccacctctttgggatggcagtagggaggtgtgctctcctggcagcacgggctgcctgcggcccttgctggacaggagaattctggaaaacaacttcattcctgtcttcagtagatctgacaggcccagaggagaaagcctgcactcttccctgtgtctgtggcactcctccaggtgtctgcatggccctctccatagtgacctatgtgtaaatgtcatcgcttctaaaagagccactctgcccagctcagctccaccactttctcttcttaccctgcttttttctcttttttagttctggaagctgaaagtacaacaggaaggtgttggcagggttggttccttctgacagctgtaaggcagggtctgttccacgcctctcccctggcttctggtggtttgctggtcctcttaggtgttccttggcttgcagatgcattatcccgacctcagccttcacgtggcgttctccccatgtgcgtttctctctgcgtcccacttcctcctttagggggtagggtgggggttcagaagaatccttcaccagctatgaggcaagtacagctaggtgggatcctggaggcttgagggagcacactgtggtggctggtctggatggtagagcgtttggtgaagcagggcacgagtcacagggaggtcgtcaggatccacgcccagctcctgcagcaggctgtggtactccggcttggtctccagcagtttcaccagattggtagactccatccgctccagctgcacctcccagtacacatagatcttctggttgaaagtgacatatacgaggcaggggctgttgcggccctctttgcaggcgtacaggcctgcacagaaggcacggatattttcatccacttggaagcggacgacggtgcggttgtgatcaatgatatatgtctgtccatcccaggcgcatgcaactacctcctcatgcccgttgccggtgacatccagtttctccagggcaaagagctggtgatccacctgcactgaccacagcagcttgtctgcttcttccatttcttccatgagcttcagtgtcccatccagggtgcacagggcaaagaggccagagccactactctcagtgccgtggccttgtttgatgttgccaattaggtgagtggagacattcttgttgtggatacggccagatgtctggtgcagcaccacgtctcgggcagctggggtctccctactaccatccgtgggcccttcagaggcaggaggggacccagtgtcctttttccaggtacacagtagaattgcatacgcacaacctggctgagacaccatcagttcaggaagacccagtggccccagagtcactgagaggctgtccacctgaccctccagcatccatttcttgagggacaccagctgccctgtcagatgttcaggaccctcacctagctcctcccagcggaaagctcgcaccacacggtctgtgtagcccaccaccagctcacgacacccatctccatcgatgtcgctgatcagcatgaccttggtgttggcagggatgtgctgcttgaagactggacgctgctcctctccgattagtgtctcgtggtgcccagaagcatccaacaccttggcaggtgtcaggtcaaacaaatgaaaccagccttcagcactcactgccaccaacaggttctttcctttattacacacgtctccaaccccaacgcaagtcagcattccctggcaggaacaggtgagccatggccgactgtcatcatttttatacacagacaccttcccgctggtgtctcccaccaccagttcatttaacgtatcgttatcaacgtctccgaggcagattgcgtgcgggaagaggctcccgctgaactccagcgccacgcgctgcacgtagctaactgacctcatggcacctccaagagcagagggagcggagaggcccagtaaatattccctgaacccccgtcgcgacagccgccagagcggaaggccacctaaggcagcaa

SEQ ID NO: 13901 - RNA, 2723 nt, Homo sapiens
  source 1..2723: mol_type = other RNA
gctgggattacaggcatgagccaccatgctcggcccagatcaactgaatttaggatttgatattactttgactttcctgcaatccaagttccttttgccagtttacttcatttgcttctgcaaatataagtacagtggtttggctttctttttaagcctttaataaaatgtctaggtgttgagactaacatcagactctttctcattaatataatacaaagccagctcgattctaattaactagttggaatttcacatgttagctctacaaatcatttttcacgcattattcctatctctataagcttgttaaaaagtgatttataaatttgttccagactctcaaagatgaagacttttgtaaacgtgtatctttggctactgtggataaaacagttgaaactccatcgcctcattaccatcatgagcatcatcacaatcatggacatcagcaccttggcagcagtgagctttcagagaatcagcaaccaggagcaccaaatgctcctactcatcctgctcctccaggccttcatcaccaccataagcacaagggtcagcataggcagggtcacccagagaaccgagatatgccagcaagtgaagatttacaagatttacaaaagaagctctgtcgaaagagatgtataaatcaattactctgtaaattgcccacagattcagagttggctcctaggagctgatgctgccattgtcgacatctgatatttgaaaaaacagggtctgcaatcacctgacagtgtaaagaaaacctcccatctttatgtagctgacagggacttcgggcagaggagaacataactgaatcttgtcagtgacgtttgcctccagctgcctgacaaataagtcagcagcttatacccacagaagccagtgccagttgacgctgaaagaatcaggcaaaaaagtgagaatgaccttcaaactaaatatttaaaataggacatactccccaatttagtctagacacaatttcatttccagcatttttataaactaccaaattagtgaaccaaaaatagaaattagatttgtgcaaacatggagaaatctactgaattggcttccagattttaaattttatgtcatagaaatattgactcaaaccatattttttatgatggagcaactgaaaggtgattgcagcttttggttaatatgtctttttttttctttttccagtgttctatttgctttaatgagaatagaaacgtaaactatgacctaggggtttctgttggataattagcagtttagaatggaggaagaacaacaaagacatgctttccatttttttctttacttatctctcaaaacaatattactttgtcttttcaatcttctacttttaactaataaaataagtggattttgtattttaagatccagaaatacttaacacgtgaatattttgctaaaaaagcatatataactattttaaatatccatttatcttttgtatatctaagactcatcctgatttttactatcacacatgaataaagcctttgtatctttctttctctaatgttgtatcatactcttctaaaacttgagtggctgtcttaaaagatataaggggaaagataatattgtctgtctctatattgcttagtaagtatttccatagtcaatgatggtttaataggtaaaccaaaccctataaacctgacctcctttatggttaatactattaagcaagaatgcagtacagaattggatacagtacggatttgtccaaataaattcaataaaaaccttaaagctgacttcgtttgttatgtaggctgtatgcatatattgaaaacagaagtgaaactttcgattgcttttaaataaataccaactaatgaatttactgctaagctcaaaaccgtctacgcttaaggtgagaatctttgccaacagaaaggcgttgctctaaatcgcgaatggtattacgaagaattgcaatctccttgtttttttcttcttgaaaatgctgaagtttccttctgtagatactttgtggcaaaacagtagaatcctgatatgattttgatttagtctgaactcttgctagtttggcatcaaattctagttgtagcttgattatttcattttgtttttctttttcttgacttcttagctttgcatttaactctgaaatttccatctcctttttctctattagttctttgtgcttttcttcatttaattcaacttttctctgcatgtcctgataaagtttgcttatttctttcttatatccctcctctttgattttcatttcacttacaagtttggcaatattattcttatattcctgttcatgagactttaacttctcttttataagatcagcacttatttttagttgttcattttcacctttcaaattctgttgatattcaatggtctgttgtagcccttttattatattatgaagagtagcacattcttctttaatggagacctcctttgcttgcattacttttaataggcaattacttttttccaactgaatatccagtatattgttctttccattggtttctaccattttcttttctatctgtgagaagtcatttataagtttgtcaagattcacactgctaatctttttcatacatccttcactgctttggtccatgcctgctgttgctcctagttccccacagtctccctttccgctgcctctggggcctggtacacccctgaat

SEQ ID NO: 13902 - RNA, 2918 nt, Homo sapiens
  source 1..2918: mol_type = other RNA
gctgggattacaggcatgagccaccatgctggccacctttggaatttctttttttttttttttttgagacagtctcactctgttgcccgggctggagtgcagtggcgcgatctcagctcactgcagcctctgcctctcaggctcaagcaattctcctgcttcagcctcccaagtagctgggattacaggcgcccaccacgatgcccagctaatttttcgtattttcagtaaagacagggtttcaccatgttggctaggctggtctcaaactcctgatccacccgcctcggcctcccaaagtgctgggattacaggcgtgaaccaccgcgcccgggtgacctttggaacttctgaccgactggcttcaagttgaggttcccacaattccctctgtaggttcaatttgctggagtggctcacaaaactaagggaaatacatttactggtttattataaaggatattataaaagatacagataaagagatgcatagggtgaggtatgaaggaagggcatggagcttcctgtgccctccctgggcgcaccacccttctagaacctctgtatgttcagttatctggaagctctctgaatccagtccccttggtttttatggaagcttcatgacagcagcattccttctagcaggatatggggtgggaccgtctctggaatgagttttatgacccaccatcagaaaggtagggaagattagagtcctgtcttgggcaggtaaaaggaagggcaggaggttagagtgattgtctcctgaggcctgacacacccaatgttgtaacaaaagagtgtaacaagggctgtgggagttatgagccaggaactgtggacgaaaatgaatgcgtgtgtttgtatatatgtgtgtctgtgtatttatatatatatgtgtgtatatacaaatacacacacacacacgccaccacaaagccaaaaaagaagaagtgatcatttttctaagtgctacgatggatgccctgggagagcgagccagagggggcatgtttatgggctgagctgcacccccccacccccaatttatgtgttgaacccctaatccccggtagctcgcaatggcccgtatgtgaatggatatggagataagagaggtgattacattaagatgaggccgtcagggggcccctcatccaatctcaccagtgtccttataagagaaaatctggacacacaaagagacaccagggacacctgcactcagaagaccaaccagggccatctccaagccaaggagagaggccttagaagaaaccaaccctgcgaacaccttggtcttggacttccagcctccaggactgtgagaaaataaatgtcttttgtttaagccactcagtctctggtattttcttatgagagccagagcagaccaacacagagggtcaggggaagcgtctatggggaggtgactcatgtactgagtcttgagggagaggtttccaggcagatggagcagcatgctccaaggccttgtgaaggaaaagagctcagtgtgctccgggaaccaggagaagatgagggaggccagggcctaaggagggcagggtaggagaggaagtggggagacatgcaggggacatgtgcacagggctgggaaggagcctgagttttcttctcagtgccatgtgaagccactgaagagttttaatgagaaaagggacataagtcagctcctattttaggaggtggcctctggctgtgtctaatggagttgacaagaataaaagtagaaggagaagaccaaggaggaggacgccaggtgagagcaggtggtggccatggagatggagaggtggagggagttaagaggcatcatggagatggaggaggcaggattgatgcaggactggggagcgtgtggtttctgcctggagcagatataggtggtgatgccctttacaaggcaagatgagcgggggtgagtggggatagccttcttgggcaggtgagggagaacagtaccatggtccaatcaacccttgcccttttgaacacatgaagctggagatgtttgtcagatgtcacaggggcagttagaacctcgagttggaacacatgggacatgtctgggctcaaaaaaatttgtgagtcaccaacacatggatgctatgtaataccaagagaatggaagagatcacctgaggagagggctcagagagaaaagtggcccaggatcagccccaaggaacagaggaggaatcagcaaagaagacagggaaggagtggctagagaagctgatagaaaacaggagagcacagtgcccgggaagcaagatgacagaccacttccggagagtggtaactgtcaattactgctgggacagagtaagacaatgcagcaaagagattgctttggatttggcaacatggaagtccctggaatccacacagaataaagctggtggcataagaatgcccctcctccaccaccactgaggaagcaccagctcccttctctttccagaggctccagctcttgacatggcaaatgtctgggctcaagttcctttctttgaactgctgttaccccacccagaattcaggaaatagaacacacagagctgctccggcagggtctctgacagcctctgcgcatagtccacgatgttgtcatgcaggtaccggctgttggtgttgagcacctggttctgctcatgtgctgcttggaccacgagagggtggcagtgcccaacgtgcgccacattgctgatgcaatcgatgtattctgccccctgttcatcgtacatgtactgcccttgggcccggacaatcttaacaggatcctcgggaaaaaagagtctgcaggaagagctgatgagccgttgcctcagggccagcgtgtcggccttcgggcgctggtctgcggccatggtgggtggccgtcagtcggt

SEQ ID NO: 13903 - RNA, 287 nt, Homo sapiens
  source 1..287: mol_type = other RNA
gctgggattacaggcatgagccaccatgctggcccttaaaattcttaactacatattttgccctataaggtaatattcagtctgttactatatatgggaatagtaatgggttctggggattaggccatgtctttttggtcaccatttagtccaccacacctagtatctctattaattagcatggcaaaattggagaacaaaaagatctctattggccagttgtggtggctcatgcctcctagtaccttaggaggccaaggctggagaatcacttgaggccaagagtt

SEQ ID NO: 13904 - RNA, 1752 nt, Homo sapiens
  source 1..1752: mol_type = other RNA
gctgggattacaggcatgagccaccatgctggcctgatacggttccttgttttaaagtgcattattcaacaagcaaagtacccgattccctttaactatgaatacaatacaaacttcgaatccagagaggtgtaaaacttgtgtgcaaagaactgtcaaggtgactttctcaaattaataaattgtcttacaatgattttctgtaaagctttctgggtctgggaaacagacctgaagtattaacacaacttgggttaattgtggaaaaagtgtcacttcaggtcacccatttccaaaagagcagcgggtcaccaaggggcccacagccacagaccggtctcagtcaaccggtctgctggctgcttttggatgagctgaagtaaaaatggattacattttaaaatacaaaattggacaccaggtgtaaacatacttgcaactgcaggcactcgagataccaggtgcctccctgttttcagcaacctaggcaagcgctaaggggtgtgctatgggtcccgcgtgctggggcagctggggtgggaaaaaccacgagaagccaagtagatactcaaggaaaacaccagaactgaagttacagagaatgaaataccagcagcacagggacagcgagagtcttttggcttttgtctgtagcttatatgagcagagtccaatatccaattaaatagatagaattcactttacgattctaattgtgctgagatccctaaaggtgaaagatccccatccttccagcagcagcagggcagcatgaagactgccaggcctcccagtcccccagcccccacatcccttggccttctggggagggggaggagctcccagaagggggaggagctcccagaacgcagcggctaaaagcctattttgcccctggtcatggagtagcccagtttcgcctcgttgttaatgaaggacatgagtcccacgtaggtctcgatgagcagggggcgctccaggatcagcacgccattcgcctgtcctggcaaagggctttctttttgggcttttttgacagcttggattaacagagccttgaagctttccaactgacacagagatgctgtcttctcatctgcgccagccatcgggtgttctgtgaaagtggcatagggcacgttggtagaccagggattccatctgtttatgaaggaaggacgactttgcttgtcccactgaattcgaatcccaaaaccttctcgcttgttgagcgatttagggggaaactggaattctccgtaggaaatggtgtctactgcgttgagcgctatccgcaccacctgctggcactggagactgatgaagtcgtatttacagataagcagggactgctccgtgaccagcaccagccgctccttctcattgttccagtgatccacctcggtaagcagccacactccctggatctcgccgtcctccacgggccgcaccaccacgcggatctcctccactgcctgctcgatgctgccgggccggaacacgaagtactccttgacgcgggcgcggcgcgtggggtcgtggatgctgagaggccagagtgtctggcgcagcggcgtccccgcccccggccgccccccgcccgggccgccgcctgcccccacctcctcgccggccgccagcaccgccgtggggctcgtaccggccgagtccaccgagtcccgcagttgcagcattgccgcaccccttaccgaccccgaccctgacgccgacgcgaccgccgtcgccgcagcc

SEQ ID NO: 13905 - RNA, 2042 nt, Homo sapiens
  source 1..2042: mol_type = other RNA
gctgggattacaggcatgagccaccatgctggctttaatccttcaaactctcactgtccttcccaggggccagtgactatgtgtatatataagtcatctgggctccaaatgagaaaagtcaaaggggcaaggatgtacagtacacagagtaggaacagagagggtcgctgaacatttttatttcaaattaggcactggaacgctggagcagctttacccactgggcggcttgtgcaggacctcaagcaatcagaatttggttatcaataaagtatttccctggttttgggagacactgagctctctgaaattaagactgtgttaaattattgttaaaatcaacaagtcccagacgctgatctttcttccccagcacatatcactatcccttttcttcttttctttttggttttcttgtttctgtctttttaatttcattatctctttaaaaatattacttcaatgcaagagccaatctagtatacatcaggaggaaaaagcagacacagtacctgtggtttttctttaagaaagtcaggtagttggaattctcccttatagacccttcgagtgttttcaataattttgggatcaggttttccgtagttaggtgggttggcatatgggtcatatccaagcttggcaagcataggagcaatcactgccatgtcttgtaaaacatctggcggtatcttcccaacccattttgatagagctcctacattgactggcttgattacttggtctgtagatctctccacttttgacagagacactcccccagctttcccaatcatctcttcatggtgcaatactgagtggttccatggaatctggaggaactttaagagtgttctcatccaccgttcaggatgtaagacaagttgttcatagtgaaccaacatgcactttttataaccaacctccatacactggttatacatggtctctatagcacgattccactttgtcaaacagtccctatagctgttcagatcaaatccagctatagtaacttttcgagaaatcattgaatgtactgatgcccggccatctcggaccatcaggagaaatttggcattggggaataacctagaaaggtaagttaaagatttcagggcaaaaggatctttattacataaataaggggctggctccccatgcttaacgataatttctagtaagaaggcttgcatggcagaatccagcacttcatcagtaacaccagcctcatccaggcggatcttctctttacttgaccgtgaccacatctgcttcagggccaggattcggggaatgaccctggtttcctctccacagcgaatgtcaggatgtgcgtccagcatggccctcatgagtgtggttccactccgaggcacacctccaataaatattaaaggcatatctttgtgataggcaaaggttttgttggctttgaggtccaggccagttctcacagtggtccttgtgctctccaatttgactggctggctacgttcctctatccggtgatggcattccatggcatgctggcccaggtaaaacacagtcacagaactaatcaccagacatgccaatagtaagttctgcttcagctttccaaccatcttgatgtggttatcttgttattaaacagatattttgctcaaaatgattttcggaaaatgttcaggccatggacagtctacttcagaaagataaccaacataacgggtaggatgatggggcgatgagctcaagaagcgcagccggggtagacgtgggggcaaatgtccgatcccggcgagacgagggtctcatcccaggggactgcggggctaggacgtggtcccagggctgggatgagtgaggagccgccgcgccgcctggacggcatcctggcctcagccgctggtcccaccgccttcggtggggggccactcgggagcccgccctcaccgccaagcgccggcagctgccagcctggaccggccccgcagagcagcgccgttccgacccgcaaccgaagccgcctcagcagcgtctcccgcggtcgccaactc

SEQ ID NO: 13906 - RNA, 1917 nt, Homo sapiens
  source 1..1917: mol_type = other RNA
gctgggattacaggcatgagccaccatgctggctttaatccttcaaactctcactgtccttcccaggggccagtgactatgtgtatatataagtcatctgggctccaaatgagaaaagtcaaaggggcaaggatgtacagtacacagagtaggaacagagagggtcgctgaacatttttatttcaaattaggcactggaacgctggagcagctttacccactgggcggcttgtgcaggacctcaagcaatcagaatttggttatcaataaagtatttccctggttttgggagacactgagctctctgaaattaagactgtgttaaattattgttaaaatcaacaagtcccagacgctgatctttcttccccagcacatatcactatcccttttcttcttttctttttggttttcttgtttctgtctttttaatttcattatctctttaaaaatattacttcaatgcaagagccaatctagtatacatcaggaggaaaaagcagacacagtacctgtggtttttctttaagaaagtcaggtagttggaattctcccttatagacccttcgagtgttttcaataattttgggatcaggttttccgtagttaggtgggttggcatatgggtcatatccaagcttggcaagcataggagcaatcactgccatgtcttgtaaaacatctggcggtatcttcccaacccattttgatagagctcctacattgactggcttgattacttggtctgtagatctctccacttttgacagagacactcccccagctttcccaatcatctcttcatggtgcaatactgagtggttccatggaatctggaggaactttaagagtgttctcatccaccgttcaggatgtaagacaagttgttcatagtgaaccaacatgcactttttataaccaacctccatacactggttatacatggtctctatagcacgattccactttgtcaaacagtccctatagctgttcagatcaaatccagctatagtaacttttcgagaaatcattgaatgtactgatgcccggccatctcggaccatcaggagaaatttggcattggggaataacctagaaaggtaagttaaagatttcagggcaaaaggatctttattacataaataaggggctggctccccatgcttaacgataatttctagtaagaaggcttgcatggcagaatccagcacttcatcagtaacaccagcctcatccaggcggatcttctctttacttgaccgtgaccacatctgcttcagggccaggattcggggaatgaccctggtttcctctccacagcgaatgtcaggatgtgcgtccagcatggccctcatgagtgtggttccactccgaggcacacctccaataaatattaaaggcatatctttgtgataggcaaaggttttgttggctttgaggtccaggccagttctcacagtggtccttgtgctctccaatttgactggctggctacgttcctctatccggtgatggcattccatggcatgctggcccaggtaaaacacagtcacagaactaatcaccagacatgccaatagtaagttctgcttcagctttccaaccatcttgatgtggttatcttgttattaaacagatattttgctcaaaatgattttcggaaaatgttcaggccatggacagtctacttcagaaagataaccaacatctgggatgagtgaggagccgccgcgccgcctggacggcatcctggcctcagccgctggtcccaccgccttcggtggggggccactcgggagcccgccctcaccgccaagcgccggcagctgccagcctggaccggccccgcagagcagcgccgttccgacccgcaaccgaagccgcctcagcagcgtctcccgcggtcgccaactcagc

SEQ ID NO: 13907 - RNA, 3809 nt, Homo sapiens
  source 1..3809: mol_type = other RNA
gctgggattacaggcatgagccaccatgcttagccaaaatagtccatcttttcaagtcagcacaagagtcctctgggacaaaaatggggaaggtccatggtgtaacttatcagaaagaaatgaaaaagcaagaagtgctgaggctactcaacaaatccttctgtgaccagatctggaattaaaaattaaagaaataaaaaagtcccagcatggtgacttatgccacgcctataatcccaacattctgggaagccaggcagaaggatcactcgagaccagcagtttgagaccagactgtgcaacacagcaagaccctgtctctacaaaaaatataaatttaaaaaatttttaaaaaggccagaagcagaggctcacactgtaatcccagcactttgggaggccaaggcaggtggatcacgaggttaggagttcaagatcagtttgaccaacatagtgaaaccccatctctactaaaagtacaaaaattacctgggtgtggtggcaggcacctgtaatcccagctactcaggaggctgagaaaggagaattgcttgaactcaggaggcagaggttgcaatgaaccaggatcacaccactgcactccagtatcggtgacagtgaaactttgtctccaaaaaaaaaaaaaaaaaaaacaaaaaaaaacaaccaaccaaccaaccaaccaaccaaacaaaaaacttaaaaaaaaaatctctcgtgaatgggagacaaccaaaatatacttctagaatacgaaataggtgaatgatgcaatgtgggtacctaccaagtagctgagatgtaatggcttttgccagataagtggcagtcacataagtctagcaagataacagggcatagtaaaaaatataatacagatgccacatgcctggagttttttcaatttgggcacatggtgccctcaaaggatctcctcccatgttacacagaaaaacataattggctgagcacagtgactcaaacctacaatctcagcactttgggaggctgaggtgtacagattgcttgagctcaggagttcgataccagcctggaaacatggtaaaaccctatatctactaatatgagaaaatagccaggcatggtggtgcatgcctgtggacccagctacatggaggctaaggtgggaagatcacttgagcctagggggcggaggatgcagtgagctacgatcgcagcactgcacaccagcatgggtgatggagtgagaccgtctctccaaaaaaaggaaaaaataataacattccctatatatctaacctatacatctacagtgtttttctcatctcagtgttctaggattcaatgacagaaggcacagtgcttttttgcaaacattacattcaaaaggcatttccgtagtgacagctctcctgtgagttttgaagccagacttctggataaatagcctatatttgccacactagtaaggccttcattcagtgttaaatataatcctgaaggaatacagaggtgtggctacaaaactgccaaatttattttacttgtaaggacttttctctggtgtgaactctccaatgtccaaggagagcagacttcttttgggtaaacattttccacatttgctgcaatcacaagatcttactcaggtgtgtgctctcctgtatttaatgagactggactcattctctgcactcataaggcctttctttcatgaactctctgatggtaacgaagtgaagagcttttcctaaattttttttcacattcactacacccataaggcttttctccagtgtgaactctcctgtgattagtgagactggagattccagcaaaagatttcccacattcactgcactcataaggcttctgaccagtgtgaactctcctgtgactagtgagataggagcttgcagcaaaagatttcccacattcactgcactcataaggcttctgaccagtgtgaactctcttatgaacaatgaatgcacagctgtgggtaaatgacttcccacaatcactgcattcatatggcctttctccagtgtgaactctctggtgtgcagtgaggtggcacttgtgcctaaaaaatttctgacaagcctcacaagcatatggcttctctccactgtgaattctctggtgtacaaggaggtgagacttcttcttaaataattttccacattcccaacacatataaggcctttttctagtatggccatgctggtgtagaatgaggttacccttgtgactaaaacatttcccacattccccacacttataaggtctttctgtagtgtgaactcgctgatgactcctaaggtgtcctttttcattaaaagatttcccacagtctccacacttgtaaggtctttctccagtgtgcatgcgctgatggatcctaaggtgcccctttgaaatataagatttcccacattctccacacttgtaaggtcttacttcagtgtgaatgcgctgatggtaactaaggctgggcttccgactaaaagatttctcacattctccacacttgtaaggtctctctccagtgtgaatgcgctgatgactcttaaggttcacgtttgaactaaaagatttcccacattctccacactcataaggcccttttccagcgtgaactttttgatggcgcctaagatatccttctaagctaaaatatttcccacattcttcacacccataaggttttcctccagtgtgaaattgctgatgttgaatgaggctgctcttttgactaaaagatttctcacattctccacattcataaggtctttttccactgtgaactctctgatgattactgaagctaacatatttgctaaaggatttcccacattcacagcacacataacattcttctcgagggagaagtctctggtgctgactgagtatatgtttggtgctaaaatgtttcatggaatctccatggctatagtgagctcccccacactgaaagggagacacacactcagttttgctgtttgacttctccccagtgtgactggcctcctgctggagtaatcctgacctgggcaaaaagtccttcccactctcactgaagacagatgactcccctgacacatgcaacttacacctcttcacaaacaacgcctcctcaacactccctctgtagggtttctctccaatgtgctcattctggtgctgatgaaagtttccactgtcatacaatttattcccccaggcctcacacctgtgcagtttctgcttgtgatgtgttccctgatgatctgccacatgcaaaatgtctcccaagatcgggccacacatctcacaggggtgggccttcttgggagacacacctgtcacaggagtcctgacctgagtctctctttgtatataaatactctgcttagaaggtgccgcctcatcttccactccacaccaacaacccagggaggacataagtgccaggttctccagagtcacatcacggtacaggcatctctgagcctcactaaggagattccattcctcctgggtaaatttcacagccacgtcttcaaaagtcactgtgccctgagcagagagcctcagcgtggccaccaccgccatcgaaccacgtggtttaaagcagggttgggaggagagggtgaccagccaggagatatgggcatgacggtccctatcctggcccaggggtgggtcacgcttggcgccgtcacagagctccagagtcgcctctgtgcagcagaggacaactgttctccgccttctgggttcagtcaccgcagtgccgacctagcgctcaggagcctctccgacaaataaacccaacaccaatc

SEQ ID NO: 13908 - RNA, 429 nt, Homo sapiens
  source 1..429: mol_type = other RNA
gctgggattacaggcatgagccaccatgcttgtccatctcctcgtttcttaaaatgagttatgcatttgtagactgatgatttatttggggcattgtcctcataaacttttcataaggcatcaatttcatcattcttcaccagaaactccatgtttgttcttgcttcaattttagcagaattcaggttgctttgataggggctcttttcaaactgtctagccttcttagtgcgtcagatccggtggaagggttctcttgcattactgacccgccaacttaatagacatccaaaattctgaggtctgggtagcttcgggttttaggtgaagggttttgttggtttgggtttggtttggttggttttctacactaaagccttccctcctccgccctttccgggtccatcggtctaatccctcccacctcgc

SEQ ID NO: 13909 - RNA, 2895 nt, Homo sapiens
  source 1..2895: mol_type = other RNA
gctgggattacaggcatgagccaccatggcccacaacattaagacagtagagatttagaggcaatgtaagtttatcgtgggtgggaatggagacgttaaatctgatggaggtatactatggaatactctgttacagtcagaaataatgaaccagagttacatacaacaacatgaagagggctgggaaatctagtattaggtgagaagggtaagaaatagagtgagatgtgatagtatgatcctatgaacacaggtttccaaaatcaactcacccagaaatagttatatattattcaaagatgtttatataaccaaggccatatatcaaacacattactcttgcctggtacctactgacaattttgcaccatgaagtagagggtgaaagggaagtggggggcagggatcaaggggaaaaagagaaaaggctactgcaaacaggagtgatgattttacaccataaaggaaaagaaagaattatcttaaccctcaaacctgttatagaactgaaatgggttctattagcccggcaccgtgagaccagatatccacatggtggtttgcaacagaagaaagtgttttattggcagggcgccaagcaaggaggctcaggtagctaagctaacgcttaaaccttgaccttccctatgactagcaggtaagggtttgtaaagcaggggtaaatttcaggaaagcagaagctataggcaaaataataaatcaatgatttatggccaaaaccataaatcaaggttacacattggttttggccttaaactgcaggatatcttgaagcaggggcttataggtcatagacagattcaaagactttctgatttgcaattggtttgagaaggtttaataatttggggtcagcagaaaagaatgttaggtccagctcatgggtgtgactttctccacgccccgcgggaagaaatttagaacaaaagatggtggtcagagttcaggtcccagatctcacttatctgaggtctacgtgcaagtggatgtgcaagcagatctgtttggtgagggttcggtttcatgttgtccaggctggtctgaaacccctgggctcaagtgatcctcctgccttggactcccaaagtgttgggattacaggtgtgagccactgtgccctcacagtccaaagctgagctgggagaaggtgggttctgctccacacagtcattcatatctccatgttttctccctagggccagtcatagtccacgtggatgaagaacgtgattggccagcctgagacgcaccccagaggcagaggagatctgatgattggtagctccatcagatgtgggaggaggagttcatgatcacaaggtcccacaacaggccatctgcaagctgaggggcaaggaaagccagtccaagtcccaaaactgaagaatcttccaaatttaatacaaaagccacatttggattttccgatgtcccaagtgtgtctaggcactgcggaacgtcgtcatgtctttgggttctctgctggggacgcaccagtcatcagcctcgtggttggtgttgtaatgcttccaggcagctttgttatacactgggagtctttctattgagtctgttgacagagccttaatgtagataactgcatctgtcccgtaaccctctagggaatacagcttcaggtctccttggaagtattgtgcgtaaagacgtgatatgggcaatccataaccaaaaccagccagaggcactgcgcgggaggtctcaacacgaggtcttggtgcagttgaatacatgtagttgaaaagtctgtcaattttcctcaaaggaacgccacctcctcggtcactcatcttcacagtcaaatcctcattacccagcgtgacatgaacttgaataggggggtaaacacctctgttggcatggtgttccatagtggctctcattgcattcttgaaaagttcaaacaccatgtgatagagatgggatggtacataaaccacttgtattggctgtcctggtgattttgcatttagttcttcaagttctagttcgggagagttaatataatacaaatcacacagacgcctagcattttcatagccatctttaataacttcaagtacattgcagtttggatttatgcttccaatgtgttttcgatgagatggacttcctttgccttttccaccaaacaataaagagtgctgattgagtaacattctaattgaaatgcgactcatgtagaatcgatccaaaaagtactgaacattctggctggtgacaggatccaccccaaagctctccttgtattcaatcacaccctgggccattgtgggaatgacatcattgtgtcggtttctgatccgtatcacagtatctgtaaagatcatcttgcaggccatacagcataaactagagacctgcaaccatgttcttctaggcctttcataaatagctttagcatcctcagcacttttgtccttaaaatcaagaagctcctgaagactctggatataccagctttgtaccaattgaacggatggtgtcctgagaagattatctggaaggagacttatttctttcattatatttgccagtctgacaggcaactcttgccgcagaaacataaatgaggtcttttcacaagcattcactgatccgaagtccaggaactgcttcatggagagcggggacggcgagaagcgcgcgtagaagtccacctggcccggaacgccgcgctcggacgccgggctggagcccgagtccgagctgaagctgcggctgaagccggcggcgcgcagccccgggcccgggccggccaaggcggctccgcgaagcagccgcgccagcctcatgccgagtcccgctagagaagccacagccagtacgccaggtttccccgcgcctctgccgagt

SEQ ID NO: 13910 - RNA, 1379 nt, Homo sapiens
  source 1..1379: mol_type = other RNA
gctgggattacaggcatgagccaccatgtcagcccataaatgatcttcggagaggtgtttcagtagaactggaataccatacggggcagaagattttgtaagcagaatatagtagtcctcccatatccgcaggggatacagtccaaaactcccagtggatgcctgaaactgacgttttagagagatcaactccatgtccagttgcctcaggatggtgttggctgcattgggactacaggaaactgctaccacatcttcctgggttaaatacatgcccttaggtggacggcacttagaacgctgagaatgatggcgatgttgtaaactctgatactctcttcttccaagtccaatcttgctagtttggacaggttgttcagtattaccctcttttttggcttcttttttgggatcataatcactatcattcccatccattggatgtgtttcttctacatcatcatcactgtcaccctgattatgtctattagctagtttacgagcctggcgatccatcaaacttgtcctagagcgagtttttttccaagaatagtaatattttacaaggcttgcaattgtcttatctggaagcatttgctgaatcctgtgaaagctctttccatgaaaactaaaggcttgttcaaataggactttatcttccactgtccactcatccggaaagggagtgaaattagggagatcagcaagggacttctcaatgttatgtttatgccagaacaacatgccaagtgcctgttccacattgtagccatgcttttcctttgcaattgcaatgtattcatccaatttggcatctgggatactgtgatatggagaccatacaagcatccctccattgtctttatctgtgtactttgtagcacctataatcccagcactttgggaggccaaggagggcggatggcttgagccccggagtttgagaccagcctgggaaacatagcaagaccttgtctctactggatcaaattcagggatccgagcttggtattcggctccgactctcatcccaacatcaccgtgctcgtcgtcgctgctgcagccgctctcgggctctgagtagtgcagcccgccgttggtggacgaggcgccgctgccgccgccgcctgccgggctcttggcgctgccgttggccgatcggttcttccccagtaactcgggccctttctccatcatgccgggcatggtagaacaggggagggggaaaggtgaggggaagaggcaggcgtcagggtgaaggcggagatggcttagagcgcgggcgggagggaaaggaggaggaggaggagacggcggcggcggcggaggaggaggaggctgttaatatggagccgccataaccgccccgctccggcagt

SEQ ID NO: 13911 - RNA, 1395 nt, Homo sapiens
  source 1..1395: mol_type = other RNA
gctgggattacaggcatgagccaccatgtcagcccataaatgatcttcggagaggtgtttcagtagaactggaataccatacggggcagaagattttgtaagcagaatatagtagtcctcccatatccgcaggggatacagtccaaaactcccagtggatgcctgaaactgacgttttagagagatcaactccatgtccagttgcctcaggatggtgttggctgcattgggactacaggaaactgctaccacatcttcctgggttaaatacatgcccttaggtggacggcacttagaacgctgagaatgatggcgatgttgtaaactctgatactctcttcttccaagtccaatcttgctagtttggacaggttgttcagtattaccctcttttttggcttcttttttgggatcataatcactatcattcccatccattggatgtgtttcttctacatcatcatcactgtcaccctgattatgtctattagctagtttacgagcctggcgatccatcaaacttgtcctagagcgagtttttttccaagaatagtaatattttacaaggcttgcaattgtcttatctggaagcatttgctgaatcctgtgaaagctctttccatgaaaactaaaggcttgttcaaataggactttatcttccactgtccactcatccggaaagggagtgaaattagggagatcagcaagggacttctcaatgttatgtttatgccagaacaacatgccaagtgcctgttccacattgtagccatgcttttcctttgcaattgcaatgtattcatccaatttggcatctgggatactgtgatatggagaccatacaagcatccctccattgtctttatctgtgtactttgtagcacctataatcccagcactttgggaggccaaggagggcggatggcttgagccccggagtttgagaccagcctgggaaacatagcaagaccttgtctctactggatcaaattcagggatccgagcttggtattcggctccgactctcatcccaacatcgtgctcgtcgtcgctgctgcagccgctctcgggctctgagtagtgcagcccgccgttggtggacgaggcgccgctgccgccgccgcctgccgggctcttggcgctgccgttggccgatcggttcttccccagtaactcgggccctttctccatcatgccgggcatggtagaacaggggagggggaaaggtgaggggaagaggcaggcgtcagggtgaaggcggagatggcttagagcgcgggcgggagggaaaggaggaggaggaggagacggcggcggcggcggaggaggaggaggctgttaatatggagccgccataaccgccccgctccggcagtagcgcagtcgcctcacaac

SEQ ID NO: 13912 - RNA, 1863 nt, Homo sapiens
  source 1..1863: mol_type = other RNA
gctgggattacaggcatgagccaccatgtccagcacactttaatattcactatgggccctcaaaaggaaatgtttgtggggccaccaaaagcaaatgtctcttgaacctagtcacctggggggacaagtgtgggaaagtgcacctgtgttcccatgagacccactcaagaggagcagaaatcctgttttgctatttccttaattgctactagggctgggattttttcatgtttattggcccctctacatttttttctttaaaaaaattcacaaagcatgtttatatttgttagctcttttgattctccctatgatagtgtgaagacagggacaaaacgctaccatttcacactcccagatctaacaatagctaccaagtaattatgccatgcgtttcttctaaccttcgcaatatcactacgaggtagttcttactatcctcattttacagataaggaaactgaggctaagtgacgctggcagacttgcccaaggccacacagctggtaacagggactggtagtcacttgagtcctacatgagcacccttgctactacagcagctcctcccctttctagaggcctagatggaaagatgctggtgtcagcggggggcacaaaggtccacccagtcccacacatgcagagaggcatcatttgttgctgataacaaagtccttggtctgcagggatgccaggtgtgggtggtgaccaaaggagcagggtccatcccatttccatctaggaagatgtgacctctgtgagtgaagagaggttctacttggctccgtgttccatcttggctccgtgttccatcccaagatgtggcatcatagacctggactgtaccatcaaaacctgagatggccaagcaattcttcaggcctggggcccaagtcactcgcagcagctctgggtcagggctaggtacggatactgggcactggactgagctcacaggatggcagagatcccgggggtcaagaagacaaagacgcccatctgagccaaggctggcaatgctgggcccagggccctggccccagctcccaacttcagcacaccatctctctccaccagacccagggccagggctgcgattctccaacggtgcccacttctgccgggtgtcaacaagccccagccggcctgaagcacagcagaaggcaaaggtgtctgcatctaggacctgcaggctactcagctcctcactgtcactgacatcattgtctgctcagctggttgggtgctggtccctgggactgcctaatcctgccccagcataggagcccttagaggccagggcttacctcttattcactgtgtatccccaacacctgaggtgtacgtggtcttccgggactccagatcaacgacctgcagacttcggagcctcgccccatggaggactccgggtgccaatgtggagaagacggccaccctaggccagagactctcctctttctcatgcacagcaatggtgctgacagctttaatgacatcactgtcctctgcaacctgccacacctgcagataacaacctggaaggccactggtaaccagcaatctggtatgtggcacatgctttagatcaaagatagacctgtctgaaaatcctccatggcgcactttgaaatctctttctgggaataagcccttgttttcctttacagaaagtctgagaggtaatttcagatgaagaatttcattctttttcaggctttcatagccagcaacaaagactcctttgtcatcaatccattcaaggactcgagtggctcctgacaggtcgaatgcatagaaatcctggtacaagcgcaaggattccaccagccagtcgtccccaggatccatggcaacgac

SEQ ID NO: 13913 - RNA, 1750 nt, Homo sapiens
  source 1..1750: mol_type = other RNA
gctgggattacaggcatgagccaccatgtccagcacactttaatattcactatgggccctcaaaaggaaatgtttgtggggccaccaaaagcaaatgtctcttgaacctagtcacctggggggacaagtgtgggaaagtgcacctgtgttcccatgagacccactcaagaggagcagaaatcctgttttgctatttccttaattgctactagggctgggattttttcatgtttattggcccctctacatttttttctttaaaaaaattcacaaagcatgtttatatttgttagctcttttgattctccctatgatagtgtgaagacagggacaaaacgctaccatttcacactcccagatctaacaatagctaccaagtaattatgccatgcgtttcttctaaccttcgcaatatcactacgaggtagttcttactatcctcattttacagataaggaaactgaggctaagtgacgctggcagacttgcccaaggccacacagctggtaacagggactggtagtcacttgagtcctacatgagcacccttgctactacagcagctcctcccctttctagaggcctagatggaaagatgctggtgtcagcggggggcacaaaggtccacccagtcccacacatgcagagaggcatcatttgttgctgataacaaagtccttggtctgcagggatgccaggtgtgggtggtgaccaaaggagcagggtccatcccatttccatctaggaagatgtgacctctgtgagtgaagagaggttctacttggctccgtgttccatcttggctccgtgttccatcccaagatgtggcatcatagacctggactgtaccatcaaaacctgagatggccaagcaattcttcaggcctggggcccaagtcactcgcagcagctctgggtcagggctaggtacggatactgggcactggactgagctcacaggatggcagagatcccgggggtcaagaagacaaagacgcccatctgagccaaggctggcaatgctgggcccagggccctggccccagctcccaacttcagcacaccatctctctccaccagacccagggccagggctgcgattctccaacggtgcccacttctgccgggtgtcaacaagccccagccggcctgaagcacagcagaaggcaaaggtgtctgcatctaggacctgcaggctactcagctcctcactgtcactgacatctgaggtgtacgtggtcttccgggactccagatcaacgacctgcagacttcggagcctcgccccatggaggactccgggtgccaatgtggagaagacggccaccctaggccagagactctcctctttctcatgcacagcaatggtgctgacagctttaatgacatcactgtcctctgcaacctgccacacctgcagataacaacctggaaggccactggtaaccagcaatctggtatgtggcacatgctttagatcaaagatagacctgtctgaaaatcctccatggcgcactttgaaatctctttctgggaataagcccttgttttcctttacagaaagtctgagaggtaatttcagatgaagaatttcattctttttcaggctttcatagccagcaacaaagactcctttgtcatcaatccattcaaggactcgagtggctcctgacaggtcgaatgcatagaaatcctggtacaagcgcaaggattccaccagccagtcgtccccaggatccatggcaacgac

SEQ ID NO: 13914 - RNA, 2284 nt, Homo sapiens
  source 1..2284: mol_type = other RNA
gctgggattacaggcatgagccaccatgtccagcacactttaatattcactatgggccctcaaaaggaaatgtttgtggggccaccaaaagcaaatgtctcttgaacctagtcacctggggggacaagtgtgggaaagtgcacctgtgttcccatgagacccactcaagaggagcagaaatcctgttttgctatttccttaattgctactagggctgggattttttcatgtttattggcccctctacatttttttctttaaaaaaattcacaaagcatgtttatatttgttagctcttttgattctccctatgatagtgtgaagacagggacaaaacgctaccatttcacactcccagatctaacaatagctaccaagtaattatgccatgcgtttcttctaaccttcgcaatatcactacgaggtagttcttactatcctcattttacagataaggaaactgaggctaagtgacgctggcagacttgcccaaggccacacagctggtaacagggactggtagtcacttgagtcctacatgagcacccttgctactacagcagctcctcccctttctagaggcctagatggaaagatgctggtgtcagcggggggcacaaaggtccacccagtcccacacatgcagagaggcatcatttgttgctgataacaaagtccttggtctgcagggatgccaggtgtgggtggtgaccaaaggagcagggtccatcccatttccatctaggaagatgtgacctctgtgagtgaagagaggttctacttggctccgtgttccatcttggctccgtgttccatcccaagatgtggcatcatagacctggactgtaccatcaaaacctgagatggccaagcaattcttcaggcctggggcccaagtcactcgcagcagctctgggtcagggctaggtacggatactgggcactggactgagctcacaggatggcagagatcccgggggtcaagaagacaaagacgcccatctgagccaaggctggcaatgctgggcccagggccctggccccagctcccaacttcagcacaccatctctctccaccagacccagggccagggctgcgattctccaacggtgcccacttctgccgggtgtcaacaagccccagccggcctgaagcacagcagaaggcaaaggtgtctgcatctaggacctgcaggctactcagctcctcactgtcactgacatctgaggtgtacgtggtcttccgggactccagatcaacgacctgcagacttcggagcctcgccccatggaggactccgggtgccaatgtggagaagacggccaccctaggccagagactctcctctttctcatgcacagcaatggtgctgacagctttaatgacatcactgtcctctgcaacctgccacacctgcagataacaacctggaaggccactggtaaccagcaatctggtatgtggcacatgctttagatcaaagatagacctgtctgaaaatcctccatggcgcactttgaaatctctttctgggaataagcccttgttttcctttacagaaagtctgagaggtaatttcagatgaagaatttcattctttttcaggctttcatagccagcaacaaagactcctttgtcatcaatccattcaaggactcgagtggctcctgacaggtcgaatgcatagaaatcctggtacctgcacaaaagggacacagaatcacacgatgcacagcacttcacagctcaaagaactccaagatggcagccgcatggttcagtggcccaaactctggagtcaggcagacgtgggactgagtttacttcccattttactccctgtttctgggaccaggccagtcccttgatgtccctgagcctcggtcctcatgtgtggacgtcccagggtacccagatttcccaaggttgacgtgaggaatcaatgagatcatctgtgttctgagctgaactcagaggctggcgcaaactaactgggcactgcgtcttcacaagcgcggctcttactagtaatctcacaacgcgcgcacgcaggaaggagccatttcctagagatgggggcctaggcccaggcggagtcctccacggtggcgagccccgaggccacagctggcccactctgcaccaggatccccaacgtgcctccacccacacccatccgcccgccaggcaagctccaggcccagctcccatgtcccagccccgtacgatttacaagcgcaaggattccaccagccagtcgtccccaggatccatggcaacgac

SEQ ID NO: 13915 - RNA, 1757 nt, Homo sapiens
  source 1..1757: mol_type = other RNA
gctgggattacaggcatgagccaccatgtccagcacactttaatattcactatgggccctcaaaaggaaatgtttgtggggccaccaaaagcaaatgtctcttgaacctagtcacctggggggacaagtgtgggaaagtgcacctgtgttcccatgagacccactcaagaggagcagaaatcctgttttgctatttccttaattgctactagggctgggattttttcatgtttattggcccctctacatttttttctttaaaaaaattcacaaagcatgtttatatttgttagctcttttgattctccctatgatagtgtgaagacagggacaaaacgctaccatttcacactcccagatctaacaatagctaccaagtaattatgccatgcgtttcttctaaccttcgcaatatcactacgaggtagttcttactatcctcattttacagataaggaaactgaggctaagtgacgctggcagacttgcccaaggccacacagctggtaacagggactggtagtcacttgagtcctacatgagcacccttgctactacagcagctcctcccctttctagaggcctagatggaaagatgctggtgtcagcggggggcacaaaggtccacccagtcccacacatgcagagaggcatcatttgttgctgataacaaagtccttggtctgcagggatgccaggtgtgggtggtgaccaaaggagcagggtccatcccatttccatctaggaagatgtgacctctgtgagtgaagagaggttctacttggctccgtgttccatcttggctccgtgttccatcccaagatgtggcatcatagacctggactgtaccatcaaaacctgagatggccaagcaattcttcaggcctggggcccaagtcactcgcagcagctctgggtcagggctaggtacggatactgggcactggactgagctcacaggatggcagagatcccgggggtcaagaagacaaagacgcccatctgagccaaggctggcaatgctgggcccagggccctggccccagctcccaacttcagcacaccatctctctccaccagacccagggccagggctgcgattctccaacggtgcccacttctgccgggtgtcaacaagccccagccggcctgaagcacagcagaaggcaaaggtgtctgcatctaggacctgcaggctactcagctcctcactgtcactgacatctgaggtgtacgtggtcttccgggactccagatcaacgacctgcagacttcggagcctcgccccatggaggactccgggtgccaatgtggagaagacggccaccctaggccagagactctcctctttctcatgcacagcaatggtgctgacagctttaatgacatcactgtcctctgcaacctgccacacctgcagataacaacctggaaggccactggtaaccagcaatctggtatgtggcacatgctttagatcaaagatagacctgtctgaaaatcctccatggcgcactttgaaatctctttctgggaataagcccttgttttcctttacagaaagtctgagaggtaatttcagatgaagaatttcattctttttcaggctttcatagccagcaacaaagactcctttgtcatcaatccattcaaggactcgagtggctcctgacaggtcgaatgcatagaaatcctggtacgatttacaagcgcaaggattccaccagccagtcgtccccaggatccatggcaacgac

SEQ ID NO: 13916 - RNA, 1661 nt, Homo sapiens
  source 1..1661: mol_type = other RNA
gctgggattacaggcatgagccaccatgtccagcacactttaatattcactatgggccctcaaaaggaaatgtttgtggggccaccaaaagcaaatgtctcttgaacctagtcacctggggggacaagtgtgggaaagtgcacctgtgttcccatgagacccactcaagaggagcagaaatcctgttttgctatttccttaattgctactagggctgggattttttcatgtttattggcccctctacatttttttctttaaaaaaattcacaaagcatgtttatatttgttagctcttttgattctccctatgatagtgtgaagacagggacaaaacgctaccatttcacactcccagatctaacaatagctaccaagtaattatgccatgcgtttcttctaaccttcgcaatatcactacgaggtagttcttactatcctcattttacagataaggaaactgaggctaagtgacgctggcagacttgcccaaggccacacagctggtaacagggactggtagtcacttgagtcctacatgagcacccttgctactacagcagctcctcccctttctagaggcctagatggaaagatgctggtgtcagcggggggcacaaaggtccacccagtcccacacatgcagagaggcatcatttgttgctgataacaaagtccttggtctgcagggatgccaggtgtgggtggtgaccaaaggagcagggtccatcccatttccatctaggaagatgtgacctctgtgagtgaagagaggttctacttggctccgtgttccatcttggctccgtgttccatcccaagatgtggcatcatagacctggactgtaccatcaaaacctgagatggccaagcaattcttcaggcctggggcccaagtcactcgcagcagctctgggtcagggctaggtacggatactgggcactggactgagctcacaggatggcagagatcccgggggtcaagaagacaaagacgcccatctgagccaaggctggcaatgctgggcccagggccctggccccagctcccaacttcagcacaccatctctctccaccagacccagggccagggctgcgattctccaacggtgcccacttctgccgggtgtcaacaagccccagccggcctgaagcacagcagaaggcaaaggtgtctgcatctaggacctgcaggctactcagctcctcactgtcactgacatctgaggtgtacgtggtcttccgggactccagatcaacgacctgcagacttcggagcctcgccccatggaggactccgggtgccaatgtggagaagacggccaccctaggccagagactctcctctttctcatgcacagcaatggtgctgacagctttaatgacatcactgtcctctgcaacctgccacacctgcagataacaacctggaaggccactggtaaccagcaatcttgttttcctttacagaaagtctgagaggtaatttcagatgaagaatttcattctttttcaggctttcatagccagcaacaaagactcctttgtcatcaatccattcaaggactcgagtggctcctgacaggtcgaatgcatagaaatcctggtacaagcgcaaggattccaccagccagtcgtccccaggatccatggcaacgac

SEQ ID NO: 13917 - RNA, 3679 nt, Homo sapiens
  source 1..3679: mol_type = other RNA
gctgggattacaggcatgagccaccatgtccagcctatttgtgctttttgaaagctccatatttaagttatatctacacatacattttaaaaagttgtatcacctatgaaagacatgtttcagtatggagagaaatagagttgggtacaataagtcactcacagcagaatgtcctggcttatgtgttagacatctgcagggcagaaaccaccagaaatctggacccactctcttctactaatcctcataagttgcatacaaggcaaattgacttgctgctttgatccaccattctgagatgggtcgtctgaatttagtctgccctaggattattcaaaaatcctgctggtgggctcctgtactatggcccctgattgatggtctttctctttcttctggacatacaagagcactcttgtttgtgggtccccttgctaaaaaatcttcccttatttttcatatggctaagcaataaacctttgaactacttatagccattggcttgagtggcgtctttagaagtctcttagaaaatagcagtcttgacaatgaactaaactagatattaacaaagtaaaatgctatttctcaataaaaatattttttccacattttcttaaattgctagatatcctgcaactcaacacctctgttctatattaaatttagattttaacttaaaacatccacacattggatacagttaaaaatactttctctactatctgatgttcactgagaagctacttcttattacatatactccataaaatataacctcatagtaaatgctttcctatagtttcctacagtttgtgcattttctctggcctcttgacttcacacagaatgattttccacattcattacacccatagggtttctgtcttatatgagttctgtggtgaacaattagagctgacttctgatgaaaggttttcccacattcattacacccaaaaggtttctccaagtgtgtcttctcaggtattctgtgaaactgtagtagtagcagaaaaatgcatcccttctcaacctagggatgctgacccaggtttcaccccgtgtgaattctctgatgtttaatgaagagtggcattgggcaaaatgtttcctatattcattcaccaataagttttttccacttttagttttgtaacatagtgtatggtccaaattccagaataatgttttcctgcattccctatcttcatattgttttttccctctttaagttctcttctatactgtgagaactgacttcagggcaaaggtgttctcattatcattatattaacagatttctctcaccctttatgttctgtgttctacaaagttctgacttcacccagagtaatttccctcgtttactacatttatagggtttctccccaagtgtattctctgatgtacagttagttttgacttaacatagaatgattttccacaaacattacattcatagggtttctcccctgtgtgtgttctatgatgtgcaatgagttttgacttcacacagaatgattttccacattgattacatccatagggtttctgtcttatatgagttctctggtgaacaattagggctgacttctgacggaaggttttcccacattcattacatccaaaaggtttctcccctgtgtgtcttctcagatgttctgtgaaaccggagtagtagcagaaaaattttccacactgaatacattcataaggtttctcacctgtgtgagttcttagatgtttagtaagggttgacttctcagagaatgacttcccacattcattacattcataaggtttttcacctgtgtgtattctttgatgtttaatgaggtctgattttctgagaaaggctttcccacatgcatagcattcatagggcttctcccctgtgtgtgttttctgatgcacagtaaggactgacttaaatgagaaggttttcccacattcatgacattcatatggtttctcccctgtgtgcgttctttgatgttgagtaagggttgacttttcactgaaggatttcccacattcatgacatccataaggtctctcccctgtatgaattctttgatgtttaatgaggtctgaattcttatagaaggtcttcccacattcatgacattcatagggttttccccctgtgtgtgttctctgatgtcttgtgtgggctgacttctgggtgaaggtttttccacattcatgacattcataaggtttttctcctgtatgtgttctctgttgtaaatgaaggactaatttttcactgaaaaatgttccacactcattatattcaataatattgttaattgagtgggttctctgaattggagtgagatttaacttctggctgaatgggtaaacactctgatgttcaaggagaatggattcctcaaagatattttctccacattcattaccatagtggttttctcttggatgtgtttgctgatgagtgatgaaaaatgacatatcacaggttttcccatgttcagtatatttgcaggttttctgtcctgtgtaacctctcttatgtacaaggaagagtgaattctcagggaaagctttcccacattcattgtattcaaaagattgttcccaatttttaattttctgatgccaaatgaggtcttcattcagccagaagctgttcccatttttattatattcagaaggttcctcttcagaatgaattatttcatgcttttcatcacagaaacattttccacctttgttaaactcattgaacttcattattgaatagtttctactggtattaattaattccagatgactctggcttggaaatttttcctctaatatccatggctcctcgcctttctccaacttgagaatcacttctggtttaggaatgcaataccctactgagacaaggtggctgtagttctccagcatcacatccctgtacagggtcctctgagcagggtccagatgctgccactcctcttgagtgaagcccacagtcacatccctaaacgacactgatccctgggatgtgatcatcttccactggtgttggaagagcagagcaaactgtgagggtgtagtctgttgtcaacgcagcaaacaccctcctgagtcctcaagcgactctgtctgttcttgactagacctttctcgcggctgtacctctgattctgtaagatcaagatgggggcatccgtacatctctagttgtgctgcagtgcgccagcagctcagcatcccacaacagctgctttgctccaagacagctgggcctaagccctttggttcgaatcctcattcaagacagaaagctcctacatcttcctgtcacttgagccatgagctggaccctctgaaaatgcccactggtgctaatggggacacaggcgaggctggacagtgccggagggcctggggtgcctccctccgcgtgcgcggcctcacaggtcagtggaaacaagaaattccccaatccacagccacgatgacttcaaaatacttcccgaagacatcaggcaatgaagctgcgaccctccgcgtcctctacccggacgccaggagatgccgggagccctccccgtcagagtgccggggagaaaaacaaacctggagccatatggcagacatgcccagaaggcccgaagcggctcccgcgacgggggccgaaaagtgcacactacatctc

SEQ ID NO: 13918 - RNA, 3590 nt, Homo sapiens
  source 1..3590: mol_type = other RNA
gctgggattacaggcatgagccaccatgtccagcctatttgtgctttttgaaagctccatatttaagttatatctacacatacattttaaaaagttgtatcacctatgaaagacatgtttcagtatggagagaaatagagttgggtacaataagtcactcacagcagaatgtcctggcttatgtgttagacatctgcagggcagaaaccaccagaaatctggacccactctcttctactaatcctcataagttgcatacaaggcaaattgacttgctgctttgatccaccattctgagatgggtcgtctgaatttagtctgccctaggattattcaaaaatcctgctggtgggctcctgtactatggcccctgattgatggtctttctctttcttctggacatacaagagcactcttgtttgtgggtccccttgctaaaaaatcttcccttatttttcatatggctaagcaataaacctttgaactacttatagccattggcttgagtggcgtctttagaagtctcttagaaaatagcagtcttgacaatgaactaaactagatattaacaaagtaaaatgctatttctcaataaaaatattttttccacattttcttaaattgctagatatcctgcaactcaacacctctgttctatattaaatttagattttaacttaaaacatccacacattggatacagttaaaaatactttctctactatctgatgttcactgagaagctacttcttattacatatactccataaaatataacctcatagtaaatgctttcctatagtttcctacagtttgtgcattttctctggcctcttgacttcacacagaatgattttccacattcattacacccatagggtttctgtcttatatgagttctgtggtgaacaattagagctgacttctgatgaaaggttttcccacattcattacacccaaaaggtttctccaagtgtgtcttctcaggtattctgtgaaactgtagtagtagcagaaaaatgcatcccttctcaacctagggatgctgacccaggtttcaccccgtgtgaattctctgatgtttaatgaagagtggcattgggcaaaatgtttcctatattcattcaccaataagttttttccacttttagttttgtaacatagtgtatggtccaaattccagaataatgttttcctgcattccctatcttcatattgttttttccctctttaagttctcttctatactgtgagaactgacttcagggcaaaggtgttctcattatcattatattaacagatttctctcaccctttatgttctgtgttctacaaagttctgacttcacccagagtaatttccctcgtttactacatttatagggtttctccccaagtgtattctctgatgtacagttagttttgacttaacatagaatgattttccacaaacattacattcatagggtttctcccctgtgtgtgttctatgatgtgcaatgagttttgacttcacacagaatgattttccacattgattacatccatagggtttctgtcttatatgagttctctggtgaacaattagggctgacttctgacggaaggttttcccacattcattacatccaaaaggtttctcccctgtgtgtcttctcagatgttctgtgaaaccggagtagtagcagaaaaattttccacactgaatacattcataaggtttctcacctgtgtgagttcttagatgtttagtaagggttgacttctcagagaatgacttcccacattcattacattcataaggtttttcacctgtgtgtattctttgatgtttaatgaggtctgattttctgagaaaggctttcccacatgcatagcattcatagggcttctcccctgtgtgtgttttctgatgcacagtaaggactgacttaaatgagaaggttttcccacattcatgacattcatatggtttctcccctgtgtgcgttctttgatgttgagtaagggttgacttttcactgaaggatttcccacattcatgacatccataaggtctctcccctgtatgaattctttgatgtttaatgaggtctgaattcttatagaaggtcttcccacattcatgacattcatagggttttccccctgtgtgtgttctctgatgtcttgtgtgggctgacttctgggtgaaggtttttccacattcatgacattcataaggtttttctcctgtatgtgttctctgttgtaaatgaaggactaatttttcactgaaaaatgttccacactcattatattcaataatattgttaattgagtgggttctctgaattggagtgagatttaacttctggctgaatgggtaaacactctgatgttcaaggagaatggattcctcaaagatattttctccacattcattaccatagtggttttctcttggatgtgtttgctgatgagtgatgaaaaatgacatatcacaggttttcccatgttcagtatatttgcaggttttctgtcctgtgtaacctctcttatgtacaaggaagagtgaattctcagggaaagctttcccacattcattgtattcaaaagattgttcccaatttttaattttctgatgccaaatgaggtcttcattcagccagaagctgttcccatttttattatattcagaaggttcctcttcagaatgaattatttcatgcttttcatcacagaaacattttccacctttgttaaactcattgaacttcattattgaatagtttctactggtattaattaattccagatgactctggcttggaaatttttcctctaatatccatggctcctcgcctttctccaacttgagaatcacttctggtttaggaatgcaataccctactgagacaaggtggctgtagttctccagcatcacatccctgtacagggtcctctgagcagggtccagatgctgccactcctcttgagtgaagcccacagtcacatccctaaacgacactgatccctgggatgtgatcatcttccactggtgttggaagagcagagcaaactgtgagggtgtagtctgttgtcaacgcagcaaacaccctcctgagtcctcaagcgactctgtctgttcttgactagacctttctcgcggctgtacctctgattctgtaagatcaagatgggggcatccgtacatctctagttgtgctgcagtgcgccagcagctcagcatcccacaacagctgctttgctccaagacagctgggcctaagccctttggttcgaatcctcattcaagacagaaagctcctacatcttcctgtcacttgagccatgagctggaccctctgaaaatgcccactggtgctaatggggacacaggcgaggctggacagtgccggagggcctggggtgcctccctccgcgtgcgcggcctcacaggtcagtggaaacaagaaattccccaatccacagccacgatgacttcaaaatacttcccgaagacatcaggcaatgaagctgcgacctggagccatatggcagacatgcccagaaggcccgaagcggctcccgcgacgggggccgaaaagt

SEQ ID NO: 13919 - RNA, 3385 nt, Homo sapiens
  source 1..3385: mol_type = other RNA
gctgggattacaggcatgagccaccatgtccagcctatttgtgctttttgaaagctccatatttaagttatatctacacatacattttaaaaagttgtatcacctatgaaagacatgtttcagtatggagagaaatagagttgggtacaataagtcactcacagcagaatgtcctggcttatgtgttagacatctgcagggcagaaaccaccagaaatctggacccactctcttctactaatcctcataagttgcatacaaggcaaattgacttgctgctttgatccaccattctgagatgggtcgtctgaatttagtctgccctaggattattcaaaaatcctgctggtgggctcctgtactatggcccctgattgatggtctttctctttcttctggacatacaagagcactcttgtttgtgggtccccttgctaaaaaatcttcccttatttttcatatggctaagcaataaacctttgaactacttatagccattggcttgagtggcgtctttagaagtctcttagaaaatagcagtcttgacaatgaactaaactagatattaacaaagtaaaatgctatttctcaataaaaatattttttccacattttcttaaattgctagatatcctgcaactcaacacctctgttctatattaaatttagattttaacttaaaacatccacacattggatacagttaaaaatactttctctactatctgatgttcactgagaagctacttcttattacatatactccataaaatataacctcatagtaaatgctttcctatagtttcctacagtttgtgcattttctctggcctcttgacttcacacagaatgattttccacattcattacacccatagggtttctgtcttatatgagttctgtggtgaacaattagagctgacttctgatgaaaggttttcccacattcattacacccaaaaggtttctccaagtgtgtcttctcaggtattctgtgaaactgtagtagtagcagaaaaatgcatcccttctcaacctagggatgctgacccaggtttcaccccgtgtgaattctctgatgtttaatgaagagtggcattgggcaaaatgtttcctatattcattcaccaataagttttttccacttttagttttgtaacatagtgtatggtccaaattccagaataatgttttcctgcattccctatcttcatattgttttttccctctttaagttctcttctatactgtgagaactgacttcagggcaaaggtgttctcattatcattatattaacagatttctctcaccctttatgttctgtgttctacaaagttctgacttcacccagagtaatttccctcgtttactacatttatagggtttctccccaagtgtattctctgatgtacagttagttttgacttaacatagaatgattttccacaaacattacattcatagggtttctcccctgtgtgtgttctatgatgtgcaatgagttttgacttcacacagaatgattttccacattgattacatccatagggtttctgtcttatatgagttctctggtgaacaattagggctgacttctgacggaaggttttcccacattcattacatccaaaaggtttctcccctgtgtgtcttctcagatgttctgtgaaaccggagtagtagcagaaaaattttccacactgaatacattcataaggtttctcacctgtgtgagttcttagatgtttagtaagggttgacttctcagagaatgacttcccacattcattacattcataaggtttttcacctgtgtgtattctttgatgtttaatgaggtctgattttctgagaaaggctttcccacatgcatagcattcatagggcttctcccctgtgtgtgttttctgatgcacagtaaggactgacttaaatgagaaggttttcccacattcatgacattcatatggtttctcccctgtgtgcgttctttgatgttgagtaagggttgacttttcactgaaggatttcccacattcatgacatccataaggtctctcccctgtatgaattctttgatgtttaatgaggtctgaattcttatagaaggtcttcccacattcatgacattcatagggttttccccctgtgtgtgttctctgatgtcttgtgtgggctgacttctgggtgaaggtttttccacattcatgacattcataaggtttttctcctgtatgtgttctctgttgtaaatgaaggactaatttttcactgaaaaatgttccacactcattatattcaataatattgttaattgagtgggttctctgaattggagtgagatttaacttctggctgaatgggtaaacactctgatgttcaaggagaatggattcctcaaagatattttctccacattcattaccatagtggttttctcttggatgtgtttgctgatgagtgatgaaaaatgacatatcacaggttttcccatgttcagtatatttgcaggttttctgtcctgtgtaacctctcttatgtacaaggaagagtgaattctcagggaaagctttcccacattcattgtattcaaaagattgttcccaatttttaattttctgatgccaaatgaggtcttcattcagccagaagctgttcccatttttattatattcagaaggttcctcttcagaatgaattatttcatgcttttcatcacagaaacattttccacctttgttaaactcattgaacttcattattgaatagtttctactggtattaattaattccagatgactctggcttggaaatttttcctctaatatccatggctcctcgcctttctccaacttgagaatcacttctggtttaggaatgcaataccctactgagacaaggtggctgtagttctccagcatcacatccctgtacagggtcctctgagcagggtccagatgctgccactcctcttgagtgaagcccacagtcacatccctaaacgacactgatccctgggatgtgatcatcttccactggtgttggaagagcagagcaaactgtgagggtgtagtctgttgtcaacgcagcaaacaccctcctgagtcctcaagcgactctgtctgttcttgactagacctttctcgcggctgtacctctgattctgtaagatcaagatgggggcatccgtacatctctagttgtgctgcagtgcgccagcagctcagcatcctccgcgtcctctacccggacgccaggagatgccgggagccctccccgtcagagtgccggggagaaaaacaaacctggagccatatggcagacatgcccagaaggcccgaagcggctcccgcgacgggggccgaaaagtgcacactacatctc

SEQ ID NO: 13920 - RNA, 3859 nt, Homo sapiens
  source 1..3859: mol_type = other RNA
gctgggattacaggcatgagccaccatgtccagcctatttgtgctttttgaaagctccatatttaagttatatctacacatacattttaaaaagttgtatcacctatgaaagacatgtttcagtatggagagaaatagagttgggtacaataagtcactcacagcagaatgtcctggcttatgtgttagacatctgcagggcagaaaccaccagaaatctggacccactctcttctactaatcctcataagttgcatacaaggcaaattgacttgctgctttgatccaccattctgagatgggtcgtctgaatttagtctgccctaggattattcaaaaatcctgctggtgggctcctgtactatggcccctgattgatggtctttctctttcttctggacatacaagagcactcttgtttgtgggtccccttgctaaaaaatcttcccttatttttcatatggctaagcaataaacctttgaactacttatagccattggcttgagtggcgtctttagaagtctcttagaaaatagcagtcttgacaatgaactaaactagatattaacaaagtaaaatgctatttctcaataaaaatattttttccacattttcttaaattgctagatatcctgcaactcaacacctctgttctatattaaatttagattttaacttaaaacatccacacattggatacagttaaaaatactttctctactatctgatgttcactgagaagctacttcttattacatatactccataaaatataacctcatagtaaatgctttcctatagtttcctacagtttgtgcattttctctggcctcttgacttcacacagaatgattttccacattcattacacccatagggtttctgtcttatatgagttctgtggtgaacaattagagctgacttctgatgaaaggttttcccacattcattacacccaaaaggtttctccaagtgtgtcttctcaggtattctgtgaaactgtagtagtagcagaaaaatgcatcccttctcaacctagggatgctgacccaggtttcaccccgtgtgaattctctgatgtttaatgaagagtggcattgggcaaaatgtttcctatattcattcaccaataagttttttccacttttagttttgtaacatagtgtatggtccaaattccagaataatgttttcctgcattccctatcttcatattgttttttccctctttaagttctcttctatactgtgagaactgacttcagggcaaaggtgttctcattatcattatattaacagatttctctcaccctttatgttctgtgttctacaaagttctgacttcacccagagtaatttccctcgtttactacatttatagggtttctccccaagtgtattctctgatgtacagttagttttgacttaacatagaatgattttccacaaacattacattcatagggtttctcccctgtgtgtgttctatgatgtgcaatgagttttgacttcacacagaatgattttccacattgattacatccatagggtttctgtcttatatgagttctctggtgaacaattagggctgacttctgacggaaggttttcccacattcattacatccaaaaggtttctcccctgtgtgtcttctcagatgttctgtgaaaccggagtagtagcagaaaaattttccacactgaatacattcataaggtttctcacctgtgtgagttcttagatgtttagtaagggttgacttctcagagaatgacttcccacattcattacattcataaggtttttcacctgtgtgtattctttgatgtttaatgaggtctgattttctgagaaaggctttcccacatgcatagcattcatagggcttctcccctgtgtgtgttttctgatgcacagtaaggactgacttaaatgagaaggttttcccacattcatgacattcatatggtttctcccctgtgtgcgttctttgatgttgagtaagggttgacttttcactgaaggatttcccacattcatgacatccataaggtctctcccctgtatgaattctttgatgtttaatgaggtctgaattcttatagaaggtcttcccacattcatgacattcatagggttttccccctgtgtgtgttctctgatgtcttgtgtgggctgacttctgggtgaaggtttttccacattcatgacattcataaggtttttctcctgtatgtgttctctgttgtaaatgaaggactaatttttcactgaaaaatgttccacactcattatattcaataatattgttaattgagtgggttctctgaattggagtgagatttaacttctggctgaatgggtaaacactctgatgttcaaggagaatggattcctcaaagatattttctccacattcattaccatagtggttttctcttggatgtgtttgctgatgagtgatgaaaaatgacatatcacaggttttcccatgttcagtatatttgcaggttttctgtcctgtgtaacctctcttatgtacaaggaagagtgaattctcagggaaagctttcccacattcattgtattcaaaagattgttcccaatttttaattttctgatgccaaatgaggtcttcattcagccagaagctgttcccatttttattatattcagaaggttcctcttcagaatgaattatttcatgcttttcatcacagaaacattttccacctttgttaaactcattgaacttcattattgaatagtttctactggtattaattaattccagatgactctggcttggaaatttttcctctaatatccatggctcctcgcctttctccaacttgagaatcacttctggtttaggaatgcaataccctactgagacaaggtggctgtagttctccagcatcacatccctgtacagggtcctctgagcagggtccagatgctgccactcctcttgagtgaagcccacagtcacatccctaaacgacactgatccctgggatgtgatcatcttccactggtgttggaagagcagagcaaactgtgagggtgtagtctgttgtcaacgcagcaaacaccctcctgagtcctcaagcgactctgtctgttcttgactagacctttctcgcggctgtacctctgattctgtaagatcaagatgggggcatccgtacatctctagttgtgctgcagtgcgccagcagctcagcatctagaacgagcgagtaacgaatccaggcatggagggtgctgtcctccacttggctgctaagctcttccctccgcatgatgccttcacaactccccaagaagcggtgctgtctgctccttcggccttgccctcttctgcccccacatctgaatgggcacaaagctcccagcctgtgggggtcccacaacagctgctttgctccaagacagctgggcctaagccctttggttcgaatcctcattcaagacagaaagctcctacatcttcctgtcacttgagccatgagctggaccctctgaaaatgcccactggtgctaatggggacacaggcgaggctggacagtgccggagggcctggggtgcctccctccgcgtgcgcggcctcacaggtcagtggaaacaagaaattccccaatccacagccacgatgacttcaaaatacttcccgaagacatcaggcaatgaagctgcgaccctccgcgtcctctacccggacgccaggagatgccgggagccctccccgtcagagtgccggggagaaaaacaaacctggagccatatggcagacatgcccagaaggcccgaagcggctcccgcgacgggggccgaaaagtgcacactacatctc

SEQ ID NO: 13921 - RNA, 3565 nt, Homo sapiens
  source 1..3565: mol_type = other RNA
gctgggattacaggcatgagccaccatgtccagcctatttgtgctttttgaaagctccatatttaagttatatctacacatacattttaaaaagttgtatcacctatgaaagacatgtttcagtatggagagaaatagagttgggtacaataagtcactcacagcagaatgtcctggcttatgtgttagacatctgcagggcagaaaccaccagaaatctggacccactctcttctactaatcctcataagttgcatacaaggcaaattgacttgctgctttgatccaccattctgagatgggtcgtctgaatttagtctgccctaggattattcaaaaatcctgctggtgggctcctgtactatggcccctgattgatggtctttctctttcttctggacatacaagagcactcttgtttgtgggtccccttgctaaaaaatcttcccttatttttcatatggctaagcaataaacctttgaactacttatagccattggcttgagtggcgtctttagaagtctcttagaaaatagcagtcttgacaatgaactaaactagatattaacaaagtaaaatgctatttctcaataaaaatattttttccacattttcttaaattgctagatatcctgcaactcaacacctctgttctatattaaatttagattttaacttaaaacatccacacattggatacagttaaaaatactttctctactatctgatgttcactgagaagctacttcttattacatatactccataaaatataacctcatagtaaatgctttcctatagtttcctacagtttgtgcattttctctggcctcttgacttcacacagaatgattttccacattcattacacccatagggtttctgtcttatatgagttctgtggtgaacaattagagctgacttctgatgaaaggttttcccacattcattacacccaaaaggtttctccaagtgtgtcttctcaggtattctgtgaaactgtagtagtagcagaaaaatgcatcccttctcaacctagggatgctgacccaggtttcaccccgtgtgaattctctgatgtttaatgaagagtggcattgggcaaaatgtttcctatattcattcaccaataagttttttccacttttagttttgtaacatagtgtatggtccaaattccagaataatgttttcctgcattccctatcttcatattgttttttccctctttaagttctcttctatactgtgagaactgacttcagggcaaaggtgttctcattatcattatattaacagatttctctcaccctttatgttctgtgttctacaaagttctgacttcacccagagtaatttccctcgtttactacatttatagggtttctccccaagtgtattctctgatgtacagttagttttgacttaacatagaatgattttccacaaacattacattcatagggtttctcccctgtgtgtgttctatgatgtgcaatgagttttgacttcacacagaatgattttccacattgattacatccatagggtttctgtcttatatgagttctctggtgaacaattagggctgacttctgacggaaggttttcccacattcattacatccaaaaggtttctcccctgtgtgtcttctcagatgttctgtgaaaccggagtagtagcagaaaaattttccacactgaatacattcataaggtttctcacctgtgtgagttcttagatgtttagtaagggttgacttctcagagaatgacttcccacattcattacattcataaggtttttcacctgtgtgtattctttgatgtttaatgaggtctgattttctgagaaaggctttcccacatgcatagcattcatagggcttctcccctgtgtgtgttttctgatgcacagtaaggactgacttaaatgagaaggttttcccacattcatgacattcatatggtttctcccctgtgtgcgttctttgatgttgagtaagggttgacttttcactgaaggatttcccacattcatgacatccataaggtctctcccctgtatgaattctttgatgtttaatgaggtctgaattcttatagaaggtcttcccacattcatgacattcatagggttttccccctgtgtgtgttctctgatgtcttgtgtgggctgacttctgggtgaaggtttttccacattcatgacattcataaggtttttctcctgtatgtgttctctgttgtaaatgaaggactaatttttcactgaaaaatgttccacactcattatattcaataatattgttaattgagtgggttctctgaattggagtgagatttaacttctggctgaatgggtaaacactctgatgttcaaggagaatggattcctcaaagatattttctccacattcattaccatagtggttttctcttggatgtgtttgctgatgagtgatgaaaaatgacatatcacaggttttcccatgttcagtatatttgcaggttttctgtcctgtgtaacctctcttatgtacaaggaagagtgaattctcagggaaagctttcccacattcattgtattcaaaagattgttcccaatttttaattttctgatgccaaatgaggtcttcattcagccagaagctgttcccatttttattatattcagaaggttcctcttcagaatgaattatttcatgcttttcatcacagaaacattttccacctttgttaaactcattgaacttcattattgaatagtttctactggtattaattaattccagatgactctggcttggaaatttttcctctaatatccatggctcctcgcctttctccaacttgagaatcacttctggtttaggaatgcaataccctactgagacaaggtggctgtagttctccagcatcacatccctgtacagggtcctctgagcagggtccagatgctgccactcctcttgagtgaagcccacagtcacatccctaaacgacactgatccctgggatgtgatcatcttccactggtgttggaagagcagagcaaactgtgagggtgtagtctgttgtcaacgcagcaaacaccctcctgagtcctcaagcgactctgtctgttcttgactagacctttctcgcggctgtacctctgattctgtaagatcaagatgggggcatccgtacatctctagttgtgctgcagtgcgccagcagctcagcatctagaacgagcgagtaacgaatccaggcatggagggtgctgtcctccacttggctgctaagctcttccctccgcatgatgccttcacaactccccaagaagcggtgctgtctgctccttcggccttgccctcttctgcccccacatctgaatgggcacaaagctcccagcctgtgggggtcctccgcgtcctctacccggacgccaggagatgccgggagccctccccgtcagagtgccggggagaaaaacaaacctggagccatatggcagacatgcccagaaggcccgaagcggctcccgcgacgggggccgaaaagtgcacactacatctc

SEQ ID NO: 13922 - RNA, 3310 nt, Homo sapiens
  source 1..3310: mol_type = other RNA
gctgggattacaggcatgagccaccatgtccagcctatttgtgctttttgaaagctccatatttaagttatatctacacatacattttaaaaagttgtatcacctatgaaagacatgtttcagtatggagagaaatagagttgggtacaataagtcactcacagcagaatgtcctggcttatgtgttagacatctgcagggcagaaaccaccagaaatctggacccactctcttctactaatcctcataagttgcatacaaggcaaattgacttgctgctttgatccaccattctgagatgggtcgtctgaatttagtctgccctaggattattcaaaaatcctgctggtgggctcctgtactatggcccctgattgatggtctttctctttcttctggacatacaagagcactcttgtttgtgggtccccttgctaaaaaatcttcccttatttttcatatggctaagcaataaacctttgaactacttatagccattggcttgagtggcgtctttagaagtctcttagaaaatagcagtcttgacaatgaactaaactagatattaacaaagtaaaatgctatttctcaataaaaatattttttccacattttcttaaattgctagatatcctgcaactcaacacctctgttctatattaaatttagattttaacttaaaacatccacacattggatacagttaaaaatactttctctactatctgatgttcactgagaagctacttcttattacatatactccataaaatataacctcatagtaaatgctttcctatagtttcctacagtttgtgcattttctctggcctcttgacttcacacagaatgattttccacattcattacacccatagggtttctgtcttatatgagttctgtggtgaacaattagagctgacttctgatgaaaggttttcccacattcattacacccaaaaggtttctccaagtgtgtcttctcaggtattctgtgaaactgtagtagtagcagaaaaatgcatcccttctcaacctagggatgctgacccaggtttcaccccgtgtgaattctctgatgtttaatgaagagtggcattgggcaaaatgtttcctatattcattcaccaataagttttttccacttttagttttgtaacatagtgtatggtccaaattccagaataatgttttcctgcattccctatcttcatattgttttttccctctttaagttctcttctatactgtgagaactgacttcagggcaaaggtgttctcattatcattatattaacagatttctctcaccctttatgttctgtgttctacaaagttctgacttcacccagagtaatttccctcgtttactacatttatagggtttctccccaagtgtattctctgatgtacagttagttttgacttaacatagaatgattttccacaaacattacattcatagggtttctcccctgtgtgtgttctatgatgtgcaatgagttttgacttcacacagaatgattttccacattgattacatccatagggtttctgtcttatatgagttctctggtgaacaattagggctgacttctgacggaaggttttcccacattcattacatccaaaaggtttctcccctgtgtgtcttctcagatgttctgtgaaaccggagtagtagcagaaaaattttccacactgaatacattcataaggtttctcacctgtgtgagttcttagatgtttagtaagggttgacttctcagagaatgacttcccacattcattacattcataaggtttttcacctgtgtgtattctttgatgtttaatgaggtctgattttctgagaaaggctttcccacatgcatagcattcatagggcttctcccctgtgtgtgttttctgatgcacagtaaggactgacttaaatgagaaggttttcccacattcatgacattcatatggtttctcccctgtgtgcgttctttgatgttgagtaagggttgacttttcactgaaggatttcccacattcatgacatccataaggtctctcccctgtatgaattctttgatgtttaatgaggtctgaattcttatagaaggtcttcccacattcatgacattcatagggttttccccctgtgtgtgttctctgatgtcttgtgtgggctgacttctgggtgaaggtttttccacattcatgacattcataaggtttttctcctgtatgtgttctctgttgtaaatgaaggactaatttttcactgaaaaatgttccacactcattatattcaataatattgttaattgagtgggttctctgaattggagtgagatttaacttctggctgaatgggtaaacactctgatgttcaaggagaatggattcctcaaagatattttctccacattcattaccatagtggttttctcttggatgtgtttgctgatgagtgatgaaaaatgacatatcacaggttttcccatgttcagtatatttgcaggttttctgtcctgtgtaacctctcttatgtacaaggaagagtgaattctcagggaaagctttcccacattcattgtattcaaaagattgttcccaatttttaattttctgatgccaaatgaggtcttcattcagccagaagctgttcccatttttattatattcagaaggttcctcttcagaatgaattatttcatgcttttcatcacagaaacattttccacctttgttaaactcattgaacttcattattgaatagtttctactggtattaattaattccagatgactctggcttggaaatttttcctctaatatccatggctcctcgcctttctccaacttgagaatcacttctggtttaggaatgcaataccctactgagacaaggtggctgtagttctccagcatcacatccctgtacagggtcctctgagcagggtccagatgctgccactcctcttgagtgaagcccacagtcacatccctaaacgacactgatccctgggatgtgatcatcttccactggtgttggaagagcagagcaaactgtgagggtgtagtctgttgtcaacgcagcaaacaccctcctgagtcctcaagcgactctgtctgttcttgactagacctttctcgcggctgtacctctgattctgtaagatcaagatgggggcatccgtacatctctagttgtgctgcagtgcgccagcagctcagcatctggagccatatggcagacatgcccagaaggcccgaagcggctcccgcgacgggggccgaaaagtgcacactacatctc

SEQ ID NO: 13923 - RNA, 3675 nt, Homo sapiens
  source 1..3675: mol_type = other RNA
gctgggattacaggcatgagccaccatgtccagcctatttgtgctttttgaaagctccatatttaagttatatctacacatacattttaaaaagttgtatcacctatgaaagacatgtttcagtatggagagaaatagagttgggtacaataagtcactcacagcagaatgtcctggcttatgtgttagacatctgcagggcagaaaccaccagaaatctggacccactctcttctactaatcctcataagttgcatacaaggcaaattgacttgctgctttgatccaccattctgagatgggtcgtctgaatttagtctgccctaggattattcaaaaatcctgctggtgggctcctgtactatggcccctgattgatggtctttctctttcttctggacatacaagagcactcttgtttgtgggtccccttgctaaaaaatcttcccttatttttcatatggctaagcaataaacctttgaactacttatagccattggcttgagtggcgtctttagaagtctcttagaaaatagcagtcttgacaatgaactaaactagatattaacaaagtaaaatgctatttctcaataaaaatattttttccacattttcttaaattgctagatatcctgcaactcaacacctctgttctatattaaatttagattttaacttaaaacatccacacattggatacagttaaaaatactttctctactatctgatgttcactgagaagctacttcttattacatatactccataaaatataacctcatagtaaatgctttcctatagtttcctacagtttgtgcattttctctggcctcttgacttcacacagaatgattttccacattcattacacccatagggtttctgtcttatatgagttctgtggtgaacaattagagctgacttctgatgaaaggttttcccacattcattacacccaaaaggtttctccaagtgtgtcttctcaggtattctgtgaaactgtagtagtagcagaaaaatgcatcccttctcaacctagggatgctgacccaggtttcaccccgtgtgaattctctgatgtttaatgaagagtggcattgggcaaaatgtttcctatattcattcaccaataagttttttccacttttagttttgtaacatagtgtatggtccaaattccagaataatgttttcctgcattccctatcttcatattgttttttccctctttaagttctcttctatactgtgagaactgacttcagggcaaaggtgttctcattatcattatattaacagatttctctcaccctttatgttctgtgttctacaaagttctgacttcacccagagtaatttccctcgtttactacatttatagggtttctccccaagtgtattctctgatgtacagttagttttgacttaacatagaatgattttccacaaacattacattcatagggtttctcccctgtgtgtgttctatgatgtgcaatgagttttgacttcacacagaatgattttccacattgattacatccatagggtttctgtcttatatgagttctctggtgaacaattagggctgacttctgacggaaggttttcccacattcattacatccaaaaggtttctcccctgtgtgtcttctcagatgttctgtgaaaccggagtagtagcagaaaaattttccacactgaatacattcataaggtttctcacctgtgtgagttcttagatgtttagtaagggttgacttctcagagaatgacttcccacattcattacattcataaggtttttcacctgtgtgtattctttgatgtttaatgaggtctgattttctgagaaaggctttcccacatgcatagcattcatagggcttctcccctgtgtgtgttttctgatgcacagtaaggactgacttaaatgagaaggttttcccacattcatgacattcatatggtttctcccctgtgtgcgttctttgatgttgagtaagggttgacttttcactgaaggatttcccacattcatgacatccataaggtctctcccctgtatgaattctttgatgtttaatgaggtctgaattcttatagaaggtcttcccacattcatgacattcatagggttttccccctgtgtgtgttctctgatgtcttgtgtgggctgacttctgggtgaaggtttttccacattcatgacattcataaggtttttctcctgtatgtgttctctgttgtaaatgaaggactaatttttcactgaaaaatgttccacactcattatattcaataatattgttaattgagtgggttctctgaattggagtgagatttaacttctggctgaatgggtaaacactctgatgttcaaggagaatggattcctcaaagatattttctccacattcattaccatagtggttttctcttggatgtgtttgctgatgagtgatgaaaaatgacatatcacaggttttcccatgttcagtatatttgcaggttttctgtcctgtgtaacctctcttatgtacaaggaagagtgaattctcagggaaagctttcccacattcattgtattcaaaagattgttcccaatttttaattttctgatgccaaatgaggtcttcattcagccagaagctgttcccatttttattatattcagaaggttcctcttcagaatgaattatttcatgcttttcatcacagaaacattttccacctttgttaaactcattgaacttcattattgaatagtttctactggtattaattaattccagatgactctggcttggaaatttttcctctaatatccatggctcctcgcctttctccaacttgagaatcacttctggtttaggaatgcaataccctactgagacaaggtggctgtagttctccagcatcacatccctgtacagggtcctctgagcagggtccagatgctgccactcctcttgagtgaagcccacagtcacatccctaaacgacactgatccctgggatgtgatcatcttccactggtgttggaagagcagagcaaactgtgagggtgtagtctgttgtcaacgcagcaaacaccctcctgagtcctcaagcgactctgtctgttcttgactctttctcgcggctgtacctctgattctgtaagatcaagatgggggcatccgtacatctctagttgtgctgcagtgcgccagcagctcagcatcccacaacagctgctttgctccaagacagctgggcctaagccctttggttcgaatcctcattcaagacagaaagctcctacatcttcctgtcacttgagccatgagctggaccctctgaaaatgcccactggtgctaatggggacacaggcgaggctggacagtgccggagggcctggggtgcctccctccgcgtgcgcggcctcacaggtcagtggaaacaagaaattccccaatccacagccacgatgacttcaaaatacttcccgaagacatcaggcaatgaagctgcgaccctccgcgtcctctacccggacgccaggagatgccgggagccctccccgtcagagtgccggggagaaaaacaaacctggagccatatggcagacatgcccagaaggcccgaagcggctcccgcgacgggggccgaaaagtgcacactacatctc

SEQ ID NO: 13924 - RNA, 3600 nt, Homo sapiens
  source 1..3600: mol_type = other RNA
gctgggattacaggcatgagccaccatgtccagcctatttgtgctttttgaaagctccatatttaagttatatctacacatacattttaaaaagttgtatcacctatgaaagacatgtttcagtatggagagaaatagagttgggtacaataagtcactcacagcagaatgtcctggcttatgtgttagacatctgcagggcagaaaccaccagaaatctggacccactctcttctactaatcctcataagttgcatacaaggcaaattgacttgctgctttgatccaccattctgagatgggtcgtctgaatttagtctgccctaggattattcaaaaatcctgctggtgggctcctgtactatggcccctgattgatggtctttctctttcttctggacatacaagagcactcttgtttgtgggtccccttgctaaaaaatcttcccttatttttcatatggctaagcaataaacctttgaactacttatagccattggcttgagtggcgtctttagaagtctcttagaaaatagcagtcttgacaatgaactaaactagatattaacaaagtaaaatgctatttctcaataaaaatattttttccacattttcttaaattgctagatatcctgcaactcaacacctctgttctatattaaatttagattttaacttaaaacatccacacattggatacagttaaaaatactttctctactatctgatgttcactgagaagctacttcttattacatatactccataaaatataacctcatagtaaatgctttcctatagtttcctacagtttgtgcattttctctggcctcttgacttcacacagaatgattttccacattcattacacccatagggtttctgtcttatatgagttctgtggtgaacaattagagctgacttctgatgaaaggttttcccacattcattacacccaaaaggtttctccaagtgtgtcttctcaggtattctgtgaaactgtagtagtagcagaaaaatgcatcccttctcaacctagggatgctgacccaggtttcaccccgtgtgaattctctgatgtttaatgaagagtggcattgggcaaaatgtttcctatattcattcaccaataagttttttccacttttagttttgtaacatagtgtatggtccaaattccagaataatgttttcctgcattccctatcttcatattgttttttccctctttaagttctcttctatactgtgagaactgacttcagggcaaaggtgttctcattatcattatattaacagatttctctcaccctttatgttctgtgttctacaaagttctgacttcacccagagtaatttccctcgtttactacatttatagggtttctccccaagtgtattctctgatgtacagttagttttgacttaacatagaatgattttccacaaacattacattcatagggtttctcccctgtgtgtgttctatgatgtgcaatgagttttgacttcacacagaatgattttccacattgattacatccatagggtttctgtcttatatgagttctctggtgaacaattagggctgacttctgacggaaggttttcccacattcattacatccaaaaggtttctcccctgtgtgtcttctcagatgttctgtgaaaccggagtagtagcagaaaaattttccacactgaatacattcataaggtttctcacctgtgtgagttcttagatgtttagtaagggttgacttctcagagaatgacttcccacattcattacattcataaggtttttcacctgtgtgtattctttgatgtttaatgaggtctgattttctgagaaaggctttcccacatgcatagcattcatagggcttctcccctgtgtgtgttttctgatgcacagtaaggactgacttaaatgagaaggttttcccacattcatgacattcatatggtttctcccctgtgtgcgttctttgatgttgagtaagggttgacttttcactgaaggatttcccacattcatgacatccataaggtctctcccctgtatgaattctttgatgtttaatgaggtctgaattcttatagaaggtcttcccacattcatgacattcatagggttttccccctgtgtgtgttctctgatgtcttgtgtgggctgacttctgggtgaaggtttttccacattcatgacattcataaggtttttctcctgtatgtgttctctgttgtaaatgaaggactaatttttcactgaaaaatgttccacactcattatattcaataatattgttaattgagtgggttctctgaattggagtgagatttaacttctggctgaatgggtaaacactctgatgttcaaggagaatggattcctcaaagatattttctccacattcattaccatagtggttttctcttggatgtgtttgctgatgagtgatgaaaaatgacatatcacaggttttcccatgttcagtatatttgcaggttttctgtcctgtgtaacctctcttatgtacaaggaagagtgaattctcagggaaagctttcccacattcattgtattcaaaagattgttcccaatttttaattttctgatgccaaatgaggtcttcattcagccagaagctgttcccatttttattatattcagaaggttcctcttcagaatgaattatttcatgcttttcatcacagaaacattttccacctttgttaaactcattgaacttcattattgaatagtttctactggtattaattaattccagatgactctggcttggaaatttttcctctaatatccatggctcctcgcctttctccaacttgagaatcacttctggtttaggaatgcaataccctactgagacaaggtggctgtagttctccagcatcacatccctgtacagggtcctctgagcagggtccagatgctgccactcctcttgagtgaagcccacagtcacatccctaaacgacactgatccctgggatgtgatcatcttccactggtgttggaagagcagagcaaactgtgagggtgtagtctgttgtcaacgcagcaaacaccctcctgagtcctcaagcgactctgtctgttcttgactctttctcgcggctgtacctctgattctgtaagatcaagatgggggcatccgtacatctctagttgtgctgcagtgcgccagcagctcagcatcccacaacagctgctttgctccaagacagctgggcctaagccctttggttcgaatcctcattcaagacagaaagctcctacatcttcctgtcacttgagccatgagctggaccctctgaaaatgcccactggtgctaatggggacacaggcgaggctggacagtgccggagggcctggggtgcctccctccgcgtgcgcggcctcacaggtcagtggaaacaagaaattccccaatccacagccacgatgacttcaaaatacttcccgaagacatcaggcaatgaagctgcgacctggagccatatggcagacatgcccagaaggcccgaagcggctcccgcgacgggggccgaaaagtgcacactacatctc

SEQ ID NO: 13925 - RNA, 3381 nt, Homo sapiens
  source 1..3381: mol_type = other RNA
gctgggattacaggcatgagccaccatgtccagcctatttgtgctttttgaaagctccatatttaagttatatctacacatacattttaaaaagttgtatcacctatgaaagacatgtttcagtatggagagaaatagagttgggtacaataagtcactcacagcagaatgtcctggcttatgtgttagacatctgcagggcagaaaccaccagaaatctggacccactctcttctactaatcctcataagttgcatacaaggcaaattgacttgctgctttgatccaccattctgagatgggtcgtctgaatttagtctgccctaggattattcaaaaatcctgctggtgggctcctgtactatggcccctgattgatggtctttctctttcttctggacatacaagagcactcttgtttgtgggtccccttgctaaaaaatcttcccttatttttcatatggctaagcaataaacctttgaactacttatagccattggcttgagtggcgtctttagaagtctcttagaaaatagcagtcttgacaatgaactaaactagatattaacaaagtaaaatgctatttctcaataaaaatattttttccacattttcttaaattgctagatatcctgcaactcaacacctctgttctatattaaatttagattttaacttaaaacatccacacattggatacagttaaaaatactttctctactatctgatgttcactgagaagctacttcttattacatatactccataaaatataacctcatagtaaatgctttcctatagtttcctacagtttgtgcattttctctggcctcttgacttcacacagaatgattttccacattcattacacccatagggtttctgtcttatatgagttctgtggtgaacaattagagctgacttctgatgaaaggttttcccacattcattacacccaaaaggtttctccaagtgtgtcttctcaggtattctgtgaaactgtagtagtagcagaaaaatgcatcccttctcaacctagggatgctgacccaggtttcaccccgtgtgaattctctgatgtttaatgaagagtggcattgggcaaaatgtttcctatattcattcaccaataagttttttccacttttagttttgtaacatagtgtatggtccaaattccagaataatgttttcctgcattccctatcttcatattgttttttccctctttaagttctcttctatactgtgagaactgacttcagggcaaaggtgttctcattatcattatattaacagatttctctcaccctttatgttctgtgttctacaaagttctgacttcacccagagtaatttccctcgtttactacatttatagggtttctccccaagtgtattctctgatgtacagttagttttgacttaacatagaatgattttccacaaacattacattcatagggtttctcccctgtgtgtgttctatgatgtgcaatgagttttgacttcacacagaatgattttccacattgattacatccatagggtttctgtcttatatgagttctctggtgaacaattagggctgacttctgacggaaggttttcccacattcattacatccaaaaggtttctcccctgtgtgtcttctcagatgttctgtgaaaccggagtagtagcagaaaaattttccacactgaatacattcataaggtttctcacctgtgtgagttcttagatgtttagtaagggttgacttctcagagaatgacttcccacattcattacattcataaggtttttcacctgtgtgtattctttgatgtttaatgaggtctgattttctgagaaaggctttcccacatgcatagcattcatagggcttctcccctgtgtgtgttttctgatgcacagtaaggactgacttaaatgagaaggttttcccacattcatgacattcatatggtttctcccctgtgtgcgttctttgatgttgagtaagggttgacttttcactgaaggatttcccacattcatgacatccataaggtctctcccctgtatgaattctttgatgtttaatgaggtctgaattcttatagaaggtcttcccacattcatgacattcatagggttttccccctgtgtgtgttctctgatgtcttgtgtgggctgacttctgggtgaaggtttttccacattcatgacattcataaggtttttctcctgtatgtgttctctgttgtaaatgaaggactaatttttcactgaaaaatgttccacactcattatattcaataatattgttaattgagtgggttctctgaattggagtgagatttaacttctggctgaatgggtaaacactctgatgttcaaggagaatggattcctcaaagatattttctccacattcattaccatagtggttttctcttggatgtgtttgctgatgagtgatgaaaaatgacatatcacaggttttcccatgttcagtatatttgcaggttttctgtcctgtgtaacctctcttatgtacaaggaagagtgaattctcagggaaagctttcccacattcattgtattcaaaagattgttcccaatttttaattttctgatgccaaatgaggtcttcattcagccagaagctgttcccatttttattatattcagaaggttcctcttcagaatgaattatttcatgcttttcatcacagaaacattttccacctttgttaaactcattgaacttcattattgaatagtttctactggtattaattaattccagatgactctggcttggaaatttttcctctaatatccatggctcctcgcctttctccaacttgagaatcacttctggtttaggaatgcaataccctactgagacaaggtggctgtagttctccagcatcacatccctgtacagggtcctctgagcagggtccagatgctgccactcctcttgagtgaagcccacagtcacatccctaaacgacactgatccctgggatgtgatcatcttccactggtgttggaagagcagagcaaactgtgagggtgtagtctgttgtcaacgcagcaaacaccctcctgagtcctcaagcgactctgtctgttcttgactctttctcgcggctgtacctctgattctgtaagatcaagatgggggcatccgtacatctctagttgtgctgcagtgcgccagcagctcagcatcctccgcgtcctctacccggacgccaggagatgccgggagccctccccgtcagagtgccggggagaaaaacaaacctggagccatatggcagacatgcccagaaggcccgaagcggctcccgcgacgggggccgaaaagtgcacactacatctc

SEQ ID NO: 13926 - RNA, 3855 nt, Homo sapiens
  source 1..3855: mol_type = other RNA
gctgggattacaggcatgagccaccatgtccagcctatttgtgctttttgaaagctccatatttaagttatatctacacatacattttaaaaagttgtatcacctatgaaagacatgtttcagtatggagagaaatagagttgggtacaataagtcactcacagcagaatgtcctggcttatgtgttagacatctgcagggcagaaaccaccagaaatctggacccactctcttctactaatcctcataagttgcatacaaggcaaattgacttgctgctttgatccaccattctgagatgggtcgtctgaatttagtctgccctaggattattcaaaaatcctgctggtgggctcctgtactatggcccctgattgatggtctttctctttcttctggacatacaagagcactcttgtttgtgggtccccttgctaaaaaatcttcccttatttttcatatggctaagcaataaacctttgaactacttatagccattggcttgagtggcgtctttagaagtctcttagaaaatagcagtcttgacaatgaactaaactagatattaacaaagtaaaatgctatttctcaataaaaatattttttccacattttcttaaattgctagatatcctgcaactcaacacctctgttctatattaaatttagattttaacttaaaacatccacacattggatacagttaaaaatactttctctactatctgatgttcactgagaagctacttcttattacatatactccataaaatataacctcatagtaaatgctttcctatagtttcctacagtttgtgcattttctctggcctcttgacttcacacagaatgattttccacattcattacacccatagggtttctgtcttatatgagttctgtggtgaacaattagagctgacttctgatgaaaggttttcccacattcattacacccaaaaggtttctccaagtgtgtcttctcaggtattctgtgaaactgtagtagtagcagaaaaatgcatcccttctcaacctagggatgctgacccaggtttcaccccgtgtgaattctctgatgtttaatgaagagtggcattgggcaaaatgtttcctatattcattcaccaataagttttttccacttttagttttgtaacatagtgtatggtccaaattccagaataatgttttcctgcattccctatcttcatattgttttttccctctttaagttctcttctatactgtgagaactgacttcagggcaaaggtgttctcattatcattatattaacagatttctctcaccctttatgttctgtgttctacaaagttctgacttcacccagagtaatttccctcgtttactacatttatagggtttctccccaagtgtattctctgatgtacagttagttttgacttaacatagaatgattttccacaaacattacattcatagggtttctcccctgtgtgtgttctatgatgtgcaatgagttttgacttcacacagaatgattttccacattgattacatccatagggtttctgtcttatatgagttctctggtgaacaattagggctgacttctgacggaaggttttcccacattcattacatccaaaaggtttctcccctgtgtgtcttctcagatgttctgtgaaaccggagtagtagcagaaaaattttccacactgaatacattcataaggtttctcacctgtgtgagttcttagatgtttagtaagggttgacttctcagagaatgacttcccacattcattacattcataaggtttttcacctgtgtgtattctttgatgtttaatgaggtctgattttctgagaaaggctttcccacatgcatagcattcatagggcttctcccctgtgtgtgttttctgatgcacagtaaggactgacttaaatgagaaggttttcccacattcatgacattcatatggtttctcccctgtgtgcgttctttgatgttgagtaagggttgacttttcactgaaggatttcccacattcatgacatccataaggtctctcccctgtatgaattctttgatgtttaatgaggtctgaattcttatagaaggtcttcccacattcatgacattcatagggttttccccctgtgtgtgttctctgatgtcttgtgtgggctgacttctgggtgaaggtttttccacattcatgacattcataaggtttttctcctgtatgtgttctctgttgtaaatgaaggactaatttttcactgaaaaatgttccacactcattatattcaataatattgttaattgagtgggttctctgaattggagtgagatttaacttctggctgaatgggtaaacactctgatgttcaaggagaatggattcctcaaagatattttctccacattcattaccatagtggttttctcttggatgtgtttgctgatgagtgatgaaaaatgacatatcacaggttttcccatgttcagtatatttgcaggttttctgtcctgtgtaacctctcttatgtacaaggaagagtgaattctcagggaaagctttcccacattcattgtattcaaaagattgttcccaatttttaattttctgatgccaaatgaggtcttcattcagccagaagctgttcccatttttattatattcagaaggttcctcttcagaatgaattatttcatgcttttcatcacagaaacattttccacctttgttaaactcattgaacttcattattgaatagtttctactggtattaattaattccagatgactctggcttggaaatttttcctctaatatccatggctcctcgcctttctccaacttgagaatcacttctggtttaggaatgcaataccctactgagacaaggtggctgtagttctccagcatcacatccctgtacagggtcctctgagcagggtccagatgctgccactcctcttgagtgaagcccacagtcacatccctaaacgacactgatccctgggatgtgatcatcttccactggtgttggaagagcagagcaaactgtgagggtgtagtctgttgtcaacgcagcaaacaccctcctgagtcctcaagcgactctgtctgttcttgactctttctcgcggctgtacctctgattctgtaagatcaagatgggggcatccgtacatctctagttgtgctgcagtgcgccagcagctcagcatctagaacgagcgagtaacgaatccaggcatggagggtgctgtcctccacttggctgctaagctcttccctccgcatgatgccttcacaactccccaagaagcggtgctgtctgctccttcggccttgccctcttctgcccccacatctgaatgggcacaaagctcccagcctgtgggggtcccacaacagctgctttgctccaagacagctgggcctaagccctttggttcgaatcctcattcaagacagaaagctcctacatcttcctgtcacttgagccatgagctggaccctctgaaaatgcccactggtgctaatggggacacaggcgaggctggacagtgccggagggcctggggtgcctccctccgcgtgcgcggcctcacaggtcagtggaaacaagaaattccccaatccacagccacgatgacttcaaaatacttcccgaagacatcaggcaatgaagctgcgaccctccgcgtcctctacccggacgccaggagatgccgggagccctccccgtcagagtgccggggagaaaaacaaacctggagccatatggcagacatgcccagaaggcccgaagcggctcccgcgacgggggccgaaaagtgcacactacatctc

SEQ ID NO: 13927 - RNA, 3768 nt, Homo sapiens
  source 1..3768: mol_type = other RNA
gctgggattacaggcatgagccaccatgtccagcctatttgtgctttttgaaagctccatatttaagttatatctacacatacattttaaaaagttgtatcacctatgaaagacatgtttcagtatggagagaaatagagttgggtacaataagtcactcacagcagaatgtcctggcttatgtgttagacatctgcagggcagaaaccaccagaaatctggacccactctcttctactaatcctcataagttgcatacaaggcaaattgacttgctgctttgatccaccattctgagatgggtcgtctgaatttagtctgccctaggattattcaaaaatcctgctggtgggctcctgtactatggcccctgattgatggtctttctctttcttctggacatacaagagcactcttgtttgtgggtccccttgctaaaaaatcttcccttatttttcatatggctaagcaataaacctttgaactacttatagccattggcttgagtggcgtctttagaagtctcttagaaaatagcagtcttgacaatgaactaaactagatattaacaaagtaaaatgctatttctcaataaaaatattttttccacattttcttaaattgctagatatcctgcaactcaacacctctgttctatattaaatttagattttaacttaaaacatccacacattggatacagttaaaaatactttctctactatctgatgttcactgagaagctacttcttattacatatactccataaaatataacctcatagtaaatgctttcctatagtttcctacagtttgtgcattttctctggcctcttgacttcacacagaatgattttccacattcattacacccatagggtttctgtcttatatgagttctgtggtgaacaattagagctgacttctgatgaaaggttttcccacattcattacacccaaaaggtttctccaagtgtgtcttctcaggtattctgtgaaactgtagtagtagcagaaaaatgcatcccttctcaacctagggatgctgacccaggtttcaccccgtgtgaattctctgatgtttaatgaagagtggcattgggcaaaatgtttcctatattcattcaccaataagttttttccacttttagttttgtaacatagtgtatggtccaaattccagaataatgttttcctgcattccctatcttcatattgttttttccctctttaagttctcttctatactgtgagaactgacttcagggcaaaggtgttctcattatcattatattaacagatttctctcaccctttatgttctgtgttctacaaagttctgacttcacccagagtaatttccctcgtttactacatttatagggtttctccccaagtgtattctctgatgtacagttagttttgacttaacatagaatgattttccacaaacattacattcatagggtttctcccctgtgtgtgttctatgatgtgcaatgagttttgacttcacacagaatgattttccacattgattacatccatagggtttctgtcttatatgagttctctggtgaacaattagggctgacttctgacggaaggttttcccacattcattacatccaaaaggtttctcccctgtgtgtcttctcagatgttctgtgaaaccggagtagtagcagaaaaattttccacactgaatacattcataaggtttctcacctgtgtgagttcttagatgtttagtaagggttgacttctcagagaatgacttcccacattcattacattcataaggtttttcacctgtgtgtattctttgatgtttaatgaggtctgattttctgagaaaggctttcccacatgcatagcattcatagggcttctcccctgtgtgtgttttctgatgcacagtaaggactgacttaaatgagaaggttttcccacattcatgacattcatatggtttctcccctgtgtgcgttctttgatgttgagtaagggttgacttttcactgaaggatttcccacattcatgacatccataaggtctctcccctgtatgaattctttgatgtttaatgaggtctgaattcttatagaaggtcttcccacattcatgacattcatagggttttccccctgtgtgtgttctctgatgtcttgtgtgggctgacttctgggtgaaggtttttccacattcatgacattcataaggtttttctcctgtatgtgttctctgttgtaaatgaaggactaatttttcactgaaaaatgttccacactcattatattcaataatattgttaattgagtgggttctctgaattggagtgagatttaacttctggctgaatgggtaaacactctgatgttcaaggagaatggattcctcaaagatattttctccacattcattaccatagtggttttctcttggatgtgtttgctgatgagtgatgaaaaatgacatatcacaggttttcccatgttcagtatatttgcaggttttctgtcctgtgtaacctctcttatgtacaaggaagagtgaattctcagggaaagctttcccacattcattgtattcaaaagattgttcccaatttttaattttctgatgccaaatgaggtcttcattcagccagaagctgttcccatttttattatattcagaaggttcctcttcagaatgaattatttcatgcttttcatcacagaaacattttccacctttgttaaactcattgaacttcattattgaatagtttctactggtattaattaattccagatgactctggcttggaaatttttcctctaatatccatggctcctcgcctttctccaacttgagaatcacttctggtttaggaatgcaataccctactgagacaaggtggctgtagttctccagcatcacatccctgtacagggtcctctgagcagggtccagatgctgccactcctcttgagtgaagcccacagtcacatccctaaacgacactgatccctgggatgtgatcatcttccactggtgttggaagagcagagcaaactgtgagggtgtagtctgttgtcaacgcagcaaacaccctcctgagtcctcaagcgactctgtctgttcttgactctttctcgcggctgtacctctgattctgtaagatcaagatgggggcatccgtacatctctagttgtgctgcagtgcgccagcagctcagcatctagaacgagcgagtaacgaatccaggcatggagggtgctgtcctccacttggctgctaagctcttccctccgcatgatgccttcacaactccccaagaagcggtgctgtctgctccttcggccttgccctcttctgcccccacatctgaatgggcacaaagctcccagcctgtgggggtcccacaacagctgctttgctccaagacagctgggcctaagccctttggttcgaatcctcattcaagacagaaagctcctacatcttcctgtcacttgagccatgagctggaccctctgaaaatgcccactggtgctaatggggacacaggcgaggctggacagtgccggagggcctggggtgcctccctccgcgtgcgcggcctcacaggtcagtggaaacaagaaattccccaatccacagccacgatgacttcaaaatacttcccgaagacatcaggcaatgaagctgcgacctggagccatatggcagacatgcccagaaggcccgaagcggctcccgcgacgggggccgaaaagtgc

SEQ ID NO: 13928 - RNA, 3561 nt, Homo sapiens
  source 1..3561: mol_type = other RNA
gctgggattacaggcatgagccaccatgtccagcctatttgtgctttttgaaagctccatatttaagttatatctacacatacattttaaaaagttgtatcacctatgaaagacatgtttcagtatggagagaaatagagttgggtacaataagtcactcacagcagaatgtcctggcttatgtgttagacatctgcagggcagaaaccaccagaaatctggacccactctcttctactaatcctcataagttgcatacaaggcaaattgacttgctgctttgatccaccattctgagatgggtcgtctgaatttagtctgccctaggattattcaaaaatcctgctggtgggctcctgtactatggcccctgattgatggtctttctctttcttctggacatacaagagcactcttgtttgtgggtccccttgctaaaaaatcttcccttatttttcatatggctaagcaataaacctttgaactacttatagccattggcttgagtggcgtctttagaagtctcttagaaaatagcagtcttgacaatgaactaaactagatattaacaaagtaaaatgctatttctcaataaaaatattttttccacattttcttaaattgctagatatcctgcaactcaacacctctgttctatattaaatttagattttaacttaaaacatccacacattggatacagttaaaaatactttctctactatctgatgttcactgagaagctacttcttattacatatactccataaaatataacctcatagtaaatgctttcctatagtttcctacagtttgtgcattttctctggcctcttgacttcacacagaatgattttccacattcattacacccatagggtttctgtcttatatgagttctgtggtgaacaattagagctgacttctgatgaaaggttttcccacattcattacacccaaaaggtttctccaagtgtgtcttctcaggtattctgtgaaactgtagtagtagcagaaaaatgcatcccttctcaacctagggatgctgacccaggtttcaccccgtgtgaattctctgatgtttaatgaagagtggcattgggcaaaatgtttcctatattcattcaccaataagttttttccacttttagttttgtaacatagtgtatggtccaaattccagaataatgttttcctgcattccctatcttcatattgttttttccctctttaagttctcttctatactgtgagaactgacttcagggcaaaggtgttctcattatcattatattaacagatttctctcaccctttatgttctgtgttctacaaagttctgacttcacccagagtaatttccctcgtttactacatttatagggtttctccccaagtgtattctctgatgtacagttagttttgacttaacatagaatgattttccacaaacattacattcatagggtttctcccctgtgtgtgttctatgatgtgcaatgagttttgacttcacacagaatgattttccacattgattacatccatagggtttctgtcttatatgagttctctggtgaacaattagggctgacttctgacggaaggttttcccacattcattacatccaaaaggtttctcccctgtgtgtcttctcagatgttctgtgaaaccggagtagtagcagaaaaattttccacactgaatacattcataaggtttctcacctgtgtgagttcttagatgtttagtaagggttgacttctcagagaatgacttcccacattcattacattcataaggtttttcacctgtgtgtattctttgatgtttaatgaggtctgattttctgagaaaggctttcccacatgcatagcattcatagggcttctcccctgtgtgtgttttctgatgcacagtaaggactgacttaaatgagaaggttttcccacattcatgacattcatatggtttctcccctgtgtgcgttctttgatgttgagtaagggttgacttttcactgaaggatttcccacattcatgacatccataaggtctctcccctgtatgaattctttgatgtttaatgaggtctgaattcttatagaaggtcttcccacattcatgacattcatagggttttccccctgtgtgtgttctctgatgtcttgtgtgggctgacttctgggtgaaggtttttccacattcatgacattcataaggtttttctcctgtatgtgttctctgttgtaaatgaaggactaatttttcactgaaaaatgttccacactcattatattcaataatattgttaattgagtgggttctctgaattggagtgagatttaacttctggctgaatgggtaaacactctgatgttcaaggagaatggattcctcaaagatattttctccacattcattaccatagtggttttctcttggatgtgtttgctgatgagtgatgaaaaatgacatatcacaggttttcccatgttcagtatatttgcaggttttctgtcctgtgtaacctctcttatgtacaaggaagagtgaattctcagggaaagctttcccacattcattgtattcaaaagattgttcccaatttttaattttctgatgccaaatgaggtcttcattcagccagaagctgttcccatttttattatattcagaaggttcctcttcagaatgaattatttcatgcttttcatcacagaaacattttccacctttgttaaactcattgaacttcattattgaatagtttctactggtattaattaattccagatgactctggcttggaaatttttcctctaatatccatggctcctcgcctttctccaacttgagaatcacttctggtttaggaatgcaataccctactgagacaaggtggctgtagttctccagcatcacatccctgtacagggtcctctgagcagggtccagatgctgccactcctcttgagtgaagcccacagtcacatccctaaacgacactgatccctgggatgtgatcatcttccactggtgttggaagagcagagcaaactgtgagggtgtagtctgttgtcaacgcagcaaacaccctcctgagtcctcaagcgactctgtctgttcttgactctttctcgcggctgtacctctgattctgtaagatcaagatgggggcatccgtacatctctagttgtgctgcagtgcgccagcagctcagcatctagaacgagcgagtaacgaatccaggcatggagggtgctgtcctccacttggctgctaagctcttccctccgcatgatgccttcacaactccccaagaagcggtgctgtctgctccttcggccttgccctcttctgcccccacatctgaatgggcacaaagctcccagcctgtgggggtcctccgcgtcctctacccggacgccaggagatgccgggagccctccccgtcagagtgccggggagaaaaacaaacctggagccatatggcagacatgcccagaaggcccgaagcggctcccgcgacgggggccgaaaagtgcacactacatctc

SEQ ID NO: 13929 - RNA, 3304 nt, Homo sapiens
  source 1..3304: mol_type = other RNA
gctgggattacaggcatgagccaccatgtccagcctatttgtgctttttgaaagctccatatttaagttatatctacacatacattttaaaaagttgtatcacctatgaaagacatgtttcagtatggagagaaatagagttgggtacaataagtcactcacagcagaatgtcctggcttatgtgttagacatctgcagggcagaaaccaccagaaatctggacccactctcttctactaatcctcataagttgcatacaaggcaaattgacttgctgctttgatccaccattctgagatgggtcgtctgaatttagtctgccctaggattattcaaaaatcctgctggtgggctcctgtactatggcccctgattgatggtctttctctttcttctggacatacaagagcactcttgtttgtgggtccccttgctaaaaaatcttcccttatttttcatatggctaagcaataaacctttgaactacttatagccattggcttgagtggcgtctttagaagtctcttagaaaatagcagtcttgacaatgaactaaactagatattaacaaagtaaaatgctatttctcaataaaaatattttttccacattttcttaaattgctagatatcctgcaactcaacacctctgttctatattaaatttagattttaacttaaaacatccacacattggatacagttaaaaatactttctctactatctgatgttcactgagaagctacttcttattacatatactccataaaatataacctcatagtaaatgctttcctatagtttcctacagtttgtgcattttctctggcctcttgacttcacacagaatgattttccacattcattacacccatagggtttctgtcttatatgagttctgtggtgaacaattagagctgacttctgatgaaaggttttcccacattcattacacccaaaaggtttctccaagtgtgtcttctcaggtattctgtgaaactgtagtagtagcagaaaaatgcatcccttctcaacctagggatgctgacccaggtttcaccccgtgtgaattctctgatgtttaatgaagagtggcattgggcaaaatgtttcctatattcattcaccaataagttttttccacttttagttttgtaacatagtgtatggtccaaattccagaataatgttttcctgcattccctatcttcatattgttttttccctctttaagttctcttctatactgtgagaactgacttcagggcaaaggtgttctcattatcattatattaacagatttctctcaccctttatgttctgtgttctacaaagttctgacttcacccagagtaatttccctcgtttactacatttatagggtttctccccaagtgtattctctgatgtacagttagttttgacttaacatagaatgattttccacaaacattacattcatagggtttctcccctgtgtgtgttctatgatgtgcaatgagttttgacttcacacagaatgattttccacattgattacatccatagggtttctgtcttatatgagttctctggtgaacaattagggctgacttctgacggaaggttttcccacattcattacatccaaaaggtttctcccctgtgtgtcttctcagatgttctgtgaaaccggagtagtagcagaaaaattttccacactgaatacattcataaggtttctcacctgtgtgagttcttagatgtttagtaagggttgacttctcagagaatgacttcccacattcattacattcataaggtttttcacctgtgtgtattctttgatgtttaatgaggtctgattttctgagaaaggctttcccacatgcatagcattcatagggcttctcccctgtgtgtgttttctgatgcacagtaaggactgacttaaatgagaaggttttcccacattcatgacattcatatggtttctcccctgtgtgcgttctttgatgttgagtaagggttgacttttcactgaaggatttcccacattcatgacatccataaggtctctcccctgtatgaattctttgatgtttaatgaggtctgaattcttatagaaggtcttcccacattcatgacattcatagggttttccccctgtgtgtgttctctgatgtcttgtgtgggctgacttctgggtgaaggtttttccacattcatgacattcataaggtttttctcctgtatgtgttctctgttgtaaatgaaggactaatttttcactgaaaaatgttccacactcattatattcaataatattgttaattgagtgggttctctgaattggagtgagatttaacttctggctgaatgggtaaacactctgatgttcaaggagaatggattcctcaaagatattttctccacattcattaccatagtggttttctcttggatgtgtttgctgatgagtgatgaaaaatgacatatcacaggttttcccatgttcagtatatttgcaggttttctgtcctgtgtaacctctcttatgtacaaggaagagtgaattctcagggaaagctttcccacattcattgtattcaaaagattgttcccaatttttaattttctgatgccaaatgaggtcttcattcagccagaagctgttcccatttttattatattcagaaggttcctcttcagaatgaattatttcatgcttttcatcacagaaacattttccacctttgttaaactcattgaacttcattattgaatagtttctactggtattaattaattccagatgactctggcttggaaatttttcctctaatatccatggctcctcgcctttctccaacttgagaatcacttctggtttaggaatgcaataccctactgagacaaggtggctgtagttctccagcatcacatccctgtacagggtcctctgagcagggtccagatgctgccactcctcttgagtgaagcccacagtcacatccctaaacgacactgatccctgggatgtgatcatcttccactggtgttggaagagcagagcaaactgtgagggtgtagtctgttgtcaacgcagcaaacaccctcctgagtcctcaagcgactctgtctgttcttgactctttctcgcggctgtacctctgattctgtaagatcaagatgggggcatccgtacatctctagttgtgctgcagtgcgccagcagctcagcatctggagccatatggcagacatgcccagaaggcccgaagcggctcccgcgacgggggccgaaaagtgcacactacatc

SEQ ID NO: 13930 - RNA, 3909 nt, Homo sapiens
  source 1..3909: mol_type = other RNA
gctgggattacaggcatgagccaccatgtccagcctatttgtgctttttgaaagctccatatttaagttatatctacacatacattttaaaaagttgtatcacctatgaaagacatgtttcagtatggagagaaatagagttgggtacaataagtcactcacagcagaatgtcctggcttatgtgttagacatctgcagggcagaaaccaccagaaatctggacccactctcttctactaatcctcataagttgcatacaaggcaaattgacttgctgctttgatccaccattctgagatgggtcgtctgaatttagtctgccctaggattattcaaaaatcctgctggtgggctcctgtactatggcccctgattgatggtctttctctttcttctggacatacaagagcactcttgtttgtgggtccccttgctaaaaaatcttcccttatttttcatatggctaagcaataaacctttgaactacttatagccattggcttgagtggcgtctttagaagtctcttagaaaatagcagtcttgacaatgaactaaactagatattaacaaagtaaaatgctatttctcaataaaaatattttttccacattttcttaaattgctagatatcctgcaactcaacacctctgttctatattaaatttagattttaacttaaaacatccacacattggatacagttaaaaatactttctctactatctgatgttcactgagaagctacttcttattacatatactccataaaatataacctcatagtaaatgctttcctatagtttcctacagtttgtgcattttctctggcctcttgacttcacacagaatgattttccacattcattacacccatagggtttctgtcttatatgagttctgtggtgaacaattagagctgacttctgatgaaaggttttcccacattcattacacccaaaaggtttctccaagtgtgtcttctcaggtattctgtgaaactgtagtagtagcagaaaaatgcatcccttctcaacctagggatgctgacccaggtttcaccccgtgtgaattctctgatgtttaatgaagagtggcattgggcaaaatgtttcctatattcattcaccaataagttttttccacttttagttttgtaacatagtgtatggtccaaattccagaataatgttttcctgcattccctatcttcatattgttttttccctctttaagttctcttctatactgtgagaactgacttcagggcaaaggtgttctcattatcattatattaacagatttctctcaccctttatgttctgtgttctacaaagttctgacttcacccagagtaatttccctcgtttactacatttatagggtttctccccaagtgtattctctgatgtacagttagttttgacttaacatagaatgattttccacaaacattacattcatagggtttctcccctgtgtgtgttctatgatgtgcaatgagttttgacttcacacagaatgattttccacattgattacatccatagggtttctgtcttatatgagttctctggtgaacaattagggctgacttctgacggaaggttttcccacattcattacatccaaaaggtttctcccctgtgtgtcttctcagatgttctgtgaaaccggagtagtagcagaaaaattttccacactgaatacattcataaggtttctcacctgtgtgagttcttagatgtttagtaagggttgacttctcagagaatgacttcccacattcattacattcataaggtttttcacctgtgtgtattctttgatgtttaatgaggtctgattttctgagaaaggctttcccacatgcatagcattcatagggcttctcccctgtgtgtgttttctgatgcacagtaaggactgacttaaatgagaaggttttcccacattcatgacattcatatggtttctcccctgtgtgcgttctttgatgttgagtaagggttgacttttcactgaaggatttcccacattcatgacatccataaggtctctcccctgtatgaattctttgatgtttaatgaggtctgaattcttatagaaggtcttcccacattcatgacattcatagggttttccccctgtgtgtgttctctgatgtcttgtgtgggctgacttctgggtgaaggtttttccacattcatgacattcataaggtttttctcctgtatgtgttctctgttgtaaatgaaggactaatttttcactgaaaaatgttccacactcattatattcaataatattgttaattgagtgggttctctgaattggagtgagatttaacttctggctgaatgggtaaacactctgatgttcaaggagaatggattcctcaaagatattttctccacattcattaccatagtggttttctcttggatgtgtttgctgatgagtgatgaaaaatgacatatcacaggttttcccatgttcagtatatttgcaggttttctgtcctgtgtaacctctcttatgtacaaggaagagtgaattctcagggaaagctttcccacattcattgtattcaaaagattgttcccaatttttaattttctgatgccaaatgaggtcttcattcagccagaagctgttcccatttttattatattcagaaggttcctcttcagaatgaattatttcatgcttttcatcacagaaacattttccacctttgttaaactcattgaacttcattattgaatagtttctactggtattaattaattcctttgtgatctaccttcctttaaattccatctggcacatactaactcacccagatgactctggcttggaaatttttcctctaatatccatggctcctcgcctttctccaacttgagaatcacttctggtttaggaatgcaataccctactgagacaaggtggctgtagttctccagcatcacatccctgtacagggtcctctgagcagggtccagatgctgccactcctcttgagtgaagcccacagtcacatccctaaacgacactgatccctgggatgtgatcatcttccactggtgttggaagagcagagcaaactgtgagggtgtagtctgttgtcaacgcagcaaacaccctcctgagtcctcaagcgactctgtctgttcttgactagacctttctcgcggctgtacctctgattctgtaagatcaagatgggggcatccgtacatctctagttgtgctgcagtgcgccagcagctcagcatctagaacgagcgagtaacgaatccaggcatggagggtgctgtcctccacttggctgctaagctcttccctccgcatgatgccttcacaactccccaagaagcggtgctgtctgctccttcggccttgccctcttctgcccccacatctgaatgggcacaaagctcccagcctgtgggggtcccacaacagctgctttgctccaagacagctgggcctaagccctttggttcgaatcctcattcaagacagaaagctcctacatcttcctgtcacttgagccatgagctggaccctctgaaaatgcccactggtgctaatggggacacaggcgaggctggacagtgccggagggcctggggtgcctccctccgcgtgcgcggcctcacaggtcagtggaaacaagaaattccccaatccacagccacgatgacttcaaaatacttcccgaagacatcaggcaatgaagctgcgaccctccgcgtcctctacccggacgccaggagatgccgggagccctccccgtcagagtgccggggagaaaaacaaacctggagccatatggcagacatgcccagaaggcccgaagcggctcccgcgacgggggccgaaaagtgcacactacatctc

SEQ ID NO: 13931 - RNA, 3431 nt, Homo sapiens
  source 1..3431: mol_type = other RNA
gctgggattacaggcatgagccaccatgtccagcctatttgtgctttttgaaagctccatatttaagttatatctacacatacattttaaaaagttgtatcacctatgaaagacatgtttcagtatggagagaaatagagttgggtacaataagtcactcacagcagaatgtcctggcttatgtgttagacatctgcagggcagaaaccaccagaaatctggacccactctcttctactaatcctcataagttgcatacaaggcaaattgacttgctgctttgatccaccattctgagatgggtcgtctgaatttagtctgccctaggattattcaaaaatcctgctggtgggctcctgtactatggcccctgattgatggtctttctctttcttctggacatacaagagcactcttgtttgtgggtccccttgctaaaaaatcttcccttatttttcatatggctaagcaataaacctttgaactacttatagccattggcttgagtggcgtctttagaagtctcttagaaaatagcagtcttgacaatgaactaaactagatattaacaaagtaaaatgctatttctcaataaaaatattttttccacattttcttaaattgctagatatcctgcaactcaacacctctgttctatattaaatttagattttaacttaaaacatccacacattggatacagttaaaaatactttctctactatctgatgttcactgagaagctacttcttattacatatactccataaaatataacctcatagtaaatgctttcctatagtttcctacagtttgtgcattttctctggcctcttgacttcacacagaatgattttccacattcattacacccatagggtttctgtcttatatgagttctgtggtgaacaattagagctgacttctgatgaaaggttttcccacattcattacacccaaaaggtttctccaagtgtgtcttctcaggtattctgtgaaactgtagtagtagcagaaaaatgcatcccttctcaacctagggatgctgacccaggtttcaccccgtgtgaattctctgatgtttaatgaagagtggcattgggcaaaatgtttcctatattcattcaccaataagttttttccacttttagttttgtaacatagtgtatggtccaaattccagaataatgttttcctgcattccctatcttcatattgttttttccctctttaagttctcttctatactgtgagaactgacttcagggcaaaggtgttctcattatcattatattaacagatttctctcaccctttatgttctgtgttctacaaagttctgacttcacccagagtaatttccctcgtttactacatttatagggtttctccccaagtgtattctctgatgtacagttagttttgacttaacatagaatgattttccacaaacattacattcatagggtttctcccctgtgtgtgttctatgatgtgcaatgagttttgacttcacacagaatgattttccacattgattacatccatagggtttctgtcttatatgagttctctggtgaacaattagggctgacttctgacggaaggttttcccacattcattacatccaaaaggtttctcccctgtgtgtcttctcagatgttctgtgaaaccggagtagtagcagaaaaattttccacactgaatacattcataaggtttctcacctgtgtgagttcttagatgtttagtaagggttgacttctcagagaatgacttcccacattcattacattcataaggtttttcacctgtgtgtattctttgatgtttaatgaggtctgattttctgagaaaggctttcccacatgcatagcattcatagggcttctcccctgtgtgtgttttctgatgcacagtaaggactgacttaaatgagaaggttttcccacattcatgacattcatatggtttctcccctgtgtgcgttctttgatgttgagtaagggttgacttttcactgaaggatttcccacattcatgacatccataaggtctctcccctgtatgaattctttgatgtttaatgaggtctgaattcttatagaaggtcttcccacattcatgacattcatagggttttccccctgtgtgtgttctctgatgtcttgtgtgggctgacttctgggtgaaggtttttccacattcatgacattcataaggtttttctcctgtatgtgttctctgttgtaaatgaaggactaatttttcactgaaaaatgttccacactcattatattcaataatattgttaattgagtgggttctctgaattggagtgagatttaacttctggctgaatgggtaaacactctgatgttcaaggagaatggattcctcaaagatattttctccacattcattaccatagtggttttctcttggatgtgtttgctgatgagtgatgaaaaatgacatatcacaggttttcccatgttcagtatatttgcaggttttctgtcctgtgtaacctctcttatgtacaaggaagagtgaattctcagggaaagctttcccacattcattgtattcaaaagattgttcccaatttttaattttctgatgccaaatgaggtcttcattcagccagaagctgttcccatttttattatattcagaaggttcctcttcagaatgaattatttcatgcttttcatcacagaaacattttccacctttgttaaactcattgaacttcattattgaatagtttctactggtattaattaattcctttgtgatctaccttcctttaaattccatctggcacatactaactcacccagatgactctggcttggaaatttttcctctaatatccatggctcctcgcctttctccaacttgagaatcacttctggtttaggaatgcaataccctactgagacaaggtggctgtagttctccagcatcacatccctgtacagggtcctctgagcagggtccagatgctgccactcctcttgagtgaagcccacagtcacatccctaaacgacactgatccctgggatgtgatcatcttccactggtgttggaagagcagagcaaactgtgagggtgtagtctgttgtcaacgcagcaaacaccctcctgagtcctcaagcgactctgtctgttcttgactctttctcgcggctgtacctctgattctgtaagatcaagatgggggcatccgtacatctctagttgtgctgcagtgcgccagcagctcagcatcctccgcgtcctctacccggacgccaggagatgccgggagccctccccgtcagagtgccggggagaaaaacaaacctggagccatatggcagacatgcccagaaggcccgaagcggctcccgcgacgggggccgaaaagtgcacactacatctc

SEQ ID NO: 13932 - RNA, 3441 nt, Homo sapiens
  source 1..3441: mol_type = other RNA
gctgggattacaggcatgagccaccatgtccagcctatttgtgctttttgaaagctccatatttaagttatatctacacatacattttaaaaagttgtatcacctatgaaagacatgtttcagtatggagagaaatagagttgggtacaataagtcactcacagcagaatgtcctggcttatgtgttagacatctgcagggcagaaaccaccagaaatctggacccactctcttctactaatcctcataagttgcatacaaggcaaattgacttgctgctttgatccaccattctgagatgggtcgtctgaatttagtctgccctaggattattcaaaaatcctgctggtgggctcctgtactatggcccctgattgatggtctttctctttcttctggacatacaagagcactcttgtttgtgggtccccttgctaaaaaatcttcccttatttttcatatggctaagcaataaacctttgaactacttatagccattggcttgagtggcgtctttagaagtctcttagaaaatagcagtcttgacaatgaactaaactagatattaacaaagtaaaatgctatttctcaataaaaatattttttccacattttcttaaattgctagatatcctgcaactcaacacctctgttctatattaaatttagattttaacttaaaacatccacacattggatacagttaaaaatactttctctactatctgatgttcactgagaagctacttcttattacatatactccataaaatataacctcatagtaaatgctttcctatagtttcctacagtttgtgcattttctctggcctcttgacttcacacagaatgattttccacattcattacacccatagggtttctgtcttatatgagttctgtggtgaacaattagagctgacttctgatgaaaggttttcccacattcattacacccaaaaggtttctccaagtgtgtcttctcaggtattctgtgaaactgtagtagtagcagaaaaatgcatcccttctcaacctagggatgctgacccaggtttcaccccgtgtgaattctctgatgtttaatgaagagtggcattgggcaaaatgtttcctatattcattcaccaataagttttttccacttttagttttgtaacatagtgtatggtccaaattccagaataatgttttcctgcattccctatcttcatattgttttttccctctttaagttctcttctatactgtgagaactgacttcagggcaaaggtgttctcattatcattatattaacagatttctctcaccctttatgttctgtgttctacaaagttctgacttcacccagagtaatttccctcgtttactacatttatagggtttctccccaagtgtattctctgatgtacagttagttttgacttaacatagaatgattttccacaaacattacattcatagggtttctcccctgtgtgtgttctatgatgtgcaatgagttttgacttcacacagaatgattttccacattgattacatccatagggtttctgtcttatatgagttctctggtgaacaattagggctgacttctgacggaaggttttcccacattcattacatccaaaaggtttctcccctgtgtgtcttctcagatgttctgtgaaaccggagtagtagcagaaaaattttccacactgaatacattcataaggtttctcacctgtgtgagttcttagatgtttagtaagggttgacttctcagagaatgacttcccacattcattacattcataaggtttttcacctgtgtgtattctttgatgtttaatgaggtctgattttctgagaaaggctttcccacatgcatagcattcatagggcttctcccctgtgtgtgttttctgatgcacagtaaggactgacttaaatgagaaggttttcccacattcatgacattcatatggtttctcccctgtgtgcgttctttgatgttgagtaagggttgacttttcactgaaggatttcccacattcatgacatccataaggtctctcccctgtatgaattctttgatgtttaatgaggtctgaattcttatagaaggtcttcccacattcatgacattcatagggttttccccctgtgtgtgttctctgatgtcttgtgtgggctgacttctgggtgaaggtttttccacattcatgacattcataaggtttttctcctgtatgtgttctctgttgtaaatgaaggactaatttttcactgaaaaatgttccacactcattatattcaataatattgttaattgagtgggttctctgaattggagtgagatttaacttctggctgaatgggtaaacactctgatgttcaaggagaatggattcctcaaagatattttctccacattcattaccatagtggttttctcttggatgtgtttgctgatgagtgatgaaaaatgacatatcacaggttttcccatgttcagtatatttgcaggttttctgtcctgtgtaacctctcttatgtacaaggaagagtgaattctcagggaaagctttcccacattcattgtattcaaaagattgttcccaatttttaattttctgatgccaaatgaggtcttcattcagccagaagctgttcccatttttattatattcagaaggttcctcttcagaatgaattatttcatgcttttcatcacagaaacattttccacctttgttaaactcattgaacttcattattgaatagtttctactggtattaattaattcctttgtgatctaccttcctttaaattccatctggcacatactaactcacccagatgactctggcttggaaatttttcctctaatatccatggctcctcgcctttctccaacttgagaatcacttctggtttaggaatgcaataccctactgagacaaggtggctgtagttctccagcatcacatccctgtacagggtcctctgagcagggtccagatgctgccactcctcttgagtgaagcccacagtcacatccctaaacgacactgatccctgggatgtgatcatcttccactggtgttggaagagcagagcaaactgtgagggtgtagtctgttgtcaacgcagcaaacaccctcctgagtcctcaagcgactctgtctgttcttgactctttctcgcggctgtacctctgattctgtaagatcaagatgggggcatccgtacatctctagttgtgctgcagtgcgccagcagctcagcatcctccgcgtcctctacccggacgccaggagatgccgggagccctccccgtcagagtgccggggagaaaaacaaacctggagccatatggcagacatgcccagaaggcccgaagcggctcccgcgacgggggccgaaaagtgcacactacatctcccacaagtcc

SEQ ID NO: 13933 - RNA, 3905 nt, Homo sapiens
  source 1..3905: mol_type = other RNA
gctgggattacaggcatgagccaccatgtccagcctatttgtgctttttgaaagctccatatttaagttatatctacacatacattttaaaaagttgtatcacctatgaaagacatgtttcagtatggagagaaatagagttgggtacaataagtcactcacagcagaatgtcctggcttatgtgttagacatctgcagggcagaaaccaccagaaatctggacccactctcttctactaatcctcataagttgcatacaaggcaaattgacttgctgctttgatccaccattctgagatgggtcgtctgaatttagtctgccctaggattattcaaaaatcctgctggtgggctcctgtactatggcccctgattgatggtctttctctttcttctggacatacaagagcactcttgtttgtgggtccccttgctaaaaaatcttcccttatttttcatatggctaagcaataaacctttgaactacttatagccattggcttgagtggcgtctttagaagtctcttagaaaatagcagtcttgacaatgaactaaactagatattaacaaagtaaaatgctatttctcaataaaaatattttttccacattttcttaaattgctagatatcctgcaactcaacacctctgttctatattaaatttagattttaacttaaaacatccacacattggatacagttaaaaatactttctctactatctgatgttcactgagaagctacttcttattacatatactccataaaatataacctcatagtaaatgctttcctatagtttcctacagtttgtgcattttctctggcctcttgacttcacacagaatgattttccacattcattacacccatagggtttctgtcttatatgagttctgtggtgaacaattagagctgacttctgatgaaaggttttcccacattcattacacccaaaaggtttctccaagtgtgtcttctcaggtattctgtgaaactgtagtagtagcagaaaaatgcatcccttctcaacctagggatgctgacccaggtttcaccccgtgtgaattctctgatgtttaatgaagagtggcattgggcaaaatgtttcctatattcattcaccaataagttttttccacttttagttttgtaacatagtgtatggtccaaattccagaataatgttttcctgcattccctatcttcatattgttttttccctctttaagttctcttctatactgtgagaactgacttcagggcaaaggtgttctcattatcattatattaacagatttctctcaccctttatgttctgtgttctacaaagttctgacttcacccagagtaatttccctcgtttactacatttatagggtttctccccaagtgtattctctgatgtacagttagttttgacttaacatagaatgattttccacaaacattacattcatagggtttctcccctgtgtgtgttctatgatgtgcaatgagttttgacttcacacagaatgattttccacattgattacatccatagggtttctgtcttatatgagttctctggtgaacaattagggctgacttctgacggaaggttttcccacattcattacatccaaaaggtttctcccctgtgtgtcttctcagatgttctgtgaaaccggagtagtagcagaaaaattttccacactgaatacattcataaggtttctcacctgtgtgagttcttagatgtttagtaagggttgacttctcagagaatgacttcccacattcattacattcataaggtttttcacctgtgtgtattctttgatgtttaatgaggtctgattttctgagaaaggctttcccacatgcatagcattcatagggcttctcccctgtgtgtgttttctgatgcacagtaaggactgacttaaatgagaaggttttcccacattcatgacattcatatggtttctcccctgtgtgcgttctttgatgttgagtaagggttgacttttcactgaaggatttcccacattcatgacatccataaggtctctcccctgtatgaattctttgatgtttaatgaggtctgaattcttatagaaggtcttcccacattcatgacattcatagggttttccccctgtgtgtgttctctgatgtcttgtgtgggctgacttctgggtgaaggtttttccacattcatgacattcataaggtttttctcctgtatgtgttctctgttgtaaatgaaggactaatttttcactgaaaaatgttccacactcattatattcaataatattgttaattgagtgggttctctgaattggagtgagatttaacttctggctgaatgggtaaacactctgatgttcaaggagaatggattcctcaaagatattttctccacattcattaccatagtggttttctcttggatgtgtttgctgatgagtgatgaaaaatgacatatcacaggttttcccatgttcagtatatttgcaggttttctgtcctgtgtaacctctcttatgtacaaggaagagtgaattctcagggaaagctttcccacattcattgtattcaaaagattgttcccaatttttaattttctgatgccaaatgaggtcttcattcagccagaagctgttcccatttttattatattcagaaggttcctcttcagaatgaattatttcatgcttttcatcacagaaacattttccacctttgttaaactcattgaacttcattattgaatagtttctactggtattaattaattcctttgtgatctaccttcctttaaattccatctggcacatactaactcacccagatgactctggcttggaaatttttcctctaatatccatggctcctcgcctttctccaacttgagaatcacttctggtttaggaatgcaataccctactgagacaaggtggctgtagttctccagcatcacatccctgtacagggtcctctgagcagggtccagatgctgccactcctcttgagtgaagcccacagtcacatccctaaacgacactgatccctgggatgtgatcatcttccactggtgttggaagagcagagcaaactgtgagggtgtagtctgttgtcaacgcagcaaacaccctcctgagtcctcaagcgactctgtctgttcttgactctttctcgcggctgtacctctgattctgtaagatcaagatgggggcatccgtacatctctagttgtgctgcagtgcgccagcagctcagcatctagaacgagcgagtaacgaatccaggcatggagggtgctgtcctccacttggctgctaagctcttccctccgcatgatgccttcacaactccccaagaagcggtgctgtctgctccttcggccttgccctcttctgcccccacatctgaatgggcacaaagctcccagcctgtgggggtcccacaacagctgctttgctccaagacagctgggcctaagccctttggttcgaatcctcattcaagacagaaagctcctacatcttcctgtcacttgagccatgagctggaccctctgaaaatgcccactggtgctaatggggacacaggcgaggctggacagtgccggagggcctggggtgcctccctccgcgtgcgcggcctcacaggtcagtggaaacaagaaattccccaatccacagccacgatgacttcaaaatacttcccgaagacatcaggcaatgaagctgcgaccctccgcgtcctctacccggacgccaggagatgccgggagccctccccgtcagagtgccggggagaaaaacaaacctggagccatatggcagacatgcccagaaggcccgaagcggctcccgcgacgggggccgaaaagtgcacactacatctc

SEQ ID NO: 13934 - RNA, 2988 nt, Homo sapiens
  source 1..2988: mol_type = other RNA
gctgggattacaggcatgagccaccatgtccagcctatttgtgctttttgaaagctccatatttaagttatatctacacatacattttaaaaagttgtatcacctatgaaagacatgtttcagtatggagagaaatagagttgggtacaataagtcactcacagcagaatgtcctggcttatgtgttagacatctgcagggcagaaaccaccagaaatctggacccactctcttctactaatcctcataagttgcatacaaggcaaattgacttgctgctttgatccaccattctgagatgggtcgtctgaatttagtctgccctaggattattcaaaaatcctgctggtgggctcctgtactatggcccctgattgatggtctttctctttcttctggacatacaagagcactcttgtttgtgggtccccttgctaaaaaatcttcccttatttttcatatggctaagcaataaacctttgaactacttatagccattggcttgagtggcgtctttagaagtctcttagaaaatagcagtcttgacaatgaactaaactagatattaacaaagtaaaatgctatttctcaataaaaatattttttccacattttcttaaattgctagatatcctgcaactcaacacctctgttctatattaaatttagattttaacttaaaacatccacacattggatacagttaaaaatactttctctactatctgatgttcactgagaagctacttcttattacatatactccataaaatataacctcatagtaaatgctttcctatagtttcctacagtttgtgcattttctctggcctcttgacttcacacagaatgattttccacattcattacacccatagggtttctgtcttatatgagttctgtggtgaacaattagagctgacttctgatgaaaggttttcccacattcattacacccaaaaggtttctccaagtgtgtcttctcaggtattctgtgaaactgtagtagtagcagaaaaatgcatcccttctcaacctagggatgctgacccaggtttcaccccgtgtgaattctctgatgtttaatgaagagtggcattgggcaaaatgtttcctatattcattcaccaataagttttttccacttttagttttgtaacatagtgtatggtccaaattccagaataatgttttcctgcattccctatcttcatattgttttttccctctttaagttctcttctatactgtgagaactgacttcagggcaaaggtgttctcattatcattatattaacagatttctctcaccctttatgttctgtgttctacaaagttctgacttcacccagagtaatttccctcgtttactacatttatagggtttctccccaagtgtattctctgatgtacagttagttttgacttaacatagaatgattttccacaaacattacattcatagggtttctcccctgtgtgtgttctatgatgtgcaatgagttttgacttcacacagaatgattttccacattgattacatccatagggtttctgtcttatatgagttctctggtgaacaattagggctgacttctgacggaaggttttcccacattcattacatccaaaaggtttctcccctgtgtgtcttctcagatgttctgtgaaaccggagtagtagcagaaaaattttccacactgaatacattcataaggtttctcacctgtgtgagttcttagatgtttagtaagggttgacttctcagagaatgacttcccacattcattacattcataaggtttttcacctgtgtgtattctttgatgtttaatgaggtctgattttctgagaaaggctttcccacatgcatagcattcatagggcttctcccctgtgtgtgttttctgatgcacagtaaggactgacttaaatgagaaggttttcccacattcatgacattcatatggtttctcccctgtgtgcgttctttgatgttgagtaagggttgacttttcactgaaggatttcccacattcatgacatccataaggtctctcccctgtatgaattctttgatgtttaatgaggtctgaattcttatagaaggtcttcccacattcatgacattcatagggttttccccctgtgtgtgttctctgatgtcttgtgtgggctgacttctgggtgaaggtttttccacattcatgacattcataaggtttttctcctgtatgtgttctctgttgtaaatgaaggactaatttttcactgaaaaatgttccacactcattatattcaataatattgttaattgagtgggttctctgaattggagtgagatttaacttctggctgaatgggtaaacactctgatgttcaaggagaatggattcctcaaagatattttctccacattcattaccatagtggttttctcttggatgtgtttgctgatgagtgatgaaaaatgacatatcacaggttttcccatgttcagtatatttgcaggttttctgtcctgtgtaacctctcttatgtacaaggaagagtgaattctcagggaaagctttcccacattcattgtattcaaaagattgttcccaatttttaattttctgatgccaaatgaggtcttcattcagccagaagctgttcccatttttattatattcagaaggttcctcttcagaatgaattatttcatgcttttcatcacagaaacattttccacctttgttaaactcattgaacttcattattgaatagtttctactggtattaattaattctatgttatgacaatgtgcacacttccagtcttatacctcttttcaagtcaacacagcagcaacaaattaaatttctaaaagttctaattcatagtcctataatccaggctccaattctgtgtggttttgttgttcttggttgttgttggtggtggtggtggtggtgtttttgagacagagtcttgctctgtcatc

SEQ ID NO: 13935 - RNA, 989 nt, Homo sapiens
  source 1..989: mol_type = other RNA
gctgggattacaggcatgagccaccatgtccagctgagactgcatttctaaaggctccaggtgaggttgctgctgtgatgctgagggtcccaggactgcatatctgctgcagggccttgccccttccaactcctgctgccttcttgacattccctcccctttcactgagcttgtgcacagactgtcttctcccctctgggctacgcacccagtttttcctgtctggaatgagctgctattcccccttaccctacacaccccatctcctctttccccaacagcaccctgtgctgaagccttcgcaggatttaccaggctgacctgttagtacctgcatggatgtcttcagagcagagactgtggattgtctatcaccaagttccagcacctggtacaggatctggcaaatcacaagccctcaggaaatatctgaaaggatgtatgcgagttaatgacatggaggtgaagagaggctcggaagggtattccaggtggagagaacggccagagcgaaggtttggaggctgaaaggcagcaacgtgcggatcttaatatctgtccttgtggtgggatgacatgagactgagagcacagctcgcggggcggggtgtcagagttccagaccttcccagtcggctcccgcagggcctcgccccggcccaggcaaggcaccaaaaccccggcccggagctctccgcgccccgagtcgccgcctcctgattggattccccctgtgtcaatccttgtcctagaacctggctgtccgttggacccgccctagagggcggggctcccgcctaggaagcgcgggggaaggtggagcgggtggaggtggggcggaaagaggatgttgaatccccacccatctggccgcagaggctccgcccaccccctttccacaggccaatacgtctgcccatcaaggccaggcgcggcctgcagtgggtgtagcaggaagggggcgggattgtgccccaggctccgccccg

SEQ ID NO: 13936 - RNA, 1986 nt, Homo sapiens
  source 1..1986: mol_type = other RNA
gctgggattacaggcatgagccaccatgtccgaccaacaatgttttaagtagttaagactgcagcatttggaaccaggggcaaatgtttgagtggtcttgagcaagttacctaaactctcaacaaagtggagactatactatattacctgattcactcagctgttatgaagactaagcaaagaaaggtacgtgaagtgcctaacccacattgtccagaatatgcaaaggcctcaacacatggatgaaaatattgcctgtctgtctgggtgcctcggttggatttattagtcaggcttgcattacagctatagaaaactccaagcagagttattgattgctcttgtagtcaacaccccataccaacaaatactttggaaacttgttggaaaaatactctttctggtagttctggactatgctcagggatcacttgggagttctagaagctgggaagaatctctcgaagctaaaagatcaaaaacaatacagggaaacacggagacgaatggatgtgagattcttccacgtgggcgaaacaagacagtcatgactaatgctagatttactcttccttggctgagagcatggtgtttattcgaagttgaatctagagtgaaagagaatatacatgtatgcaaaacatcataagggagagttgtcttaaagacagtggctcctcatctcaaattcattagcatatacatgcccacacaagaacacaaaagaactttctgccccaaccaattaaaaatatcaaaaaggagaaatgaaaacagattttctgtcttaccaaaatattatttttattactttcatttcctaggttatgggtgttaataaatgctaaaagcatttctaaatctagaaatccatcccacaagatgtttttctagagtccacaaaaatcacacagttatgttaatttgcgagtaaggaaactatgaacaacagaggtagagttaatatgagtagagaaagggtctaacaccaagtggcacaaatgcaattaaatcctggttcacgtgacccccccaattcacaactttacttttatcaacatcccaccattcaggaaacttttagcgcactaaattcctttattttgtgaaaaaaattatcatgtgaaatgactgctatataggacagtcaattaaatttgagtgtcaaaaactgactttctttaaacatagcaaaaccctccaaaggtaagcaatctaaaagtatttttttcttgatcagtaagtctaaactctgctattaacaccatctatcaggttctcatgatgacattgcaagcaatgccagaactagagcccaggtggctatgactcaacaactgggtatcattggcagaaagaaagaaatctgaggtttcaaaatggaatgagaaaggaaatgaaggccactttccccttactccacaatgaatgaagtattgatactgggactcacctggtgcaagaatgaagaaacagctggattttatttgttccttttgcctgctccttagaacaatggaacctgcactaaccagcttcacaaagagctttgattgatggcagcttttcagatacctctgtggcttagtcttatcttgtttggtatctctattgtttctgaacccagaattttttccataagggcacgtcactatcacttgatagacttttcccaccaggctcttttctttccacgctttctgaagtagatatgctgctcaatgatggagtttcaccagggatccaggctgaacaccctctcacagggccacctcctgatctttagttctgtgagcctttgctgtttcgtgctagagcttttagttgaaagtaaaatgaaagaagtcctcagacttcatgaattccaggtgtctgtgaagtgggactggcaacattttttcctcccaccataaaaaagttctctagtcggagaaagtattctgaagcttctctgttcagaccctggtgttctgaaacacactgaga

SEQ ID NO: 13937 - RNA, 10102 nt, Homo sapiens
  source 1..10102: mol_type = other RNA
gctgggattacaggcatgagccaccatgtccggccctcttaacattcttgctctttctgttttcaaacagagaaagccagctccaagaagtcaggaaacaacaaggctgagctagcctccgcttcacagcaggtatgtggaggagctttgactgccctccgaggggcagaatagaagcttcttgaggaacactgatctttcactagtctacccaatgtgtcagcctcccctgccagcaaacaccatgtagaaataatgaataaagatgcatagaaaacaggaaaacccaagagccagtcctacaactgtcacttcccaatgacttggccttgagcaagttccattgcccttgagctctgttcgggtcccctatgtgtaaaggtgtgtttggttctccctctgacacagggttggggaccaagtacatccaggctgacaggtcctggtgatgaatagggtgtaccatatatagtgacattgatgcagattatgcatgtgtgtgttttatattttgaagtgaaattgacataagacaaaatcactttgaagtgaacgattcagaagcgttcagtgcattcacaatgtgagtaatgaccacctctacctagttcaaaaacattttcagtgccccaaaataaacccccatggccactaagcagtcattccccattccctactctcaccaacctctggcaacctggaaactgcttcctatctctatggatttacctatcctgagcattccccataagtggaattatatgatatgagacctcttgtctcttgactttcactaacacgtttgaggttcatccaagttgtagcatctgcacttcgtccctttttacggttgaataatattccattatgtacataccgcaatttgtttatccattcatccagtaatgggcagctgagatgtttccgccttttggttatcacgaataatgttgcggtagacattcatgtagcaggtgacgtcttttaaggcactttcacatttcattctaacaagtatgtgaggtagaccctggtcatatgaatggcatttgagctgtgcttccttcctcattaagccatcactttctaatcccaccccacttttataataagaaaaacaatgaagaacttctaaggctaagtcgggcacatgaagcgtttgtgaaggaataaaaaggtattgattaataatttgatttttaaaaattaatcataactcagaatgtgtaacaggactgtctcaaaactggacattattcctaacatgcatggaaaatgcaaagatggtattaaagattaaattctttaaaaagtaaagacactgcagggacatggaaagaaaaatgatacaggaaagaccaaagcaaagctcttcatctccaaatctttgccatctaatttagtgaccagaacactcagacctttctttgaacagagccatttttatcaagtcaagatctcacgaccatccaaagactctgagctcaaaacctcatgtggacagacgcaaatgtgaggcaacctggccagccttctgctgctctgctacaggtctgggcaaatgaaagaacgtgctcaaatctaaactcaggtaatggagaggctaatgttgtcaacatcaatattgtcactgcttccaagacaacttctcagcaaaacaaagagtctcaactccctctaggtgttaagaatcttcaagtatcaagtgaaaaggtctccgttcccttgaattcttttttaatccaaggtttggggcttcaaattcagtataaagcgagtgcaatcacagtaggttacttgaaggggcaaaatgcaatctcaccttaggagccaggcctgccagacccagtcccatcaatcagccagccacgggcacaaaacacacgctgatgaaaaggacttggcactgtgcattgtgtcatgtccaatactcgtcattgtatacataataaagtcagtcagatgaacattctcatactgtgttccccatgtgatgcaaaaaataacaaaattggactattgagaattttaaaggcacacagaaaaaaaagggagtgctaagcctacaaattctctggctggaatgataccaaagtcctccttctcatggtctccacgatcaccaattgttcatttctctcttttgtcttccccaatcaagaccctcagttcaggggtacacaaatcaggaggaggcagggagaaaattttttttaagattaatcttgaacacttaaattttaccaaaggcaaggaaaaggtaagaggaaatatattttctacctctacctccacacccctagcccttccctcccaagggtactttgctttaaagtgaaatcagggacattctgccaggaaaggtcatttagtaaacatgtcaggctttgagggccctttggtctctgctgtgactactcacctatgccactgtagcataaaagtaaccacagacaaaacccaaatgaatgggctgtgttcccataaaactttagggatgcactcttacatttgaaattcataccatttttgcatgtcacaaaacattactgttttcatttttttccccaactctttaatagtcattcttagctcatgggccaatagcaggctgcatttggcccagaggctgtagtctgcctaccccttctttaaatcatggatgctaactttttaggatatggtgtatctggtttttttctttatttataggggagggaggtttaaagttctgcataaaccggaaaagaacaaggcaaggacattacaacagcatatttcagaaagaaaatacctacccctgttctgtgaatctcaagaaaatttaaagagtcctttagtcacctgttggcagaggaccacaaattttaaaatatgcttgcttactgctaaaagttaaatgtttcattcctttctctttgataaaagaaattcaagcatagttactcctattttctgaatcaaatcagtaagtactcactagatgcctctaacgtgtctagtactggtcatgctgccagaaagaaaggacatcaaaatatatcttttcccccaaacattttgatccccgagagattttagtgttatagcttcagtatgaaggtgacaaattgagactgatccctcccaaaccatgatctcagctgatcccctttcatccactgaatgcattttagagatgagtttggccagtggatagtatacatatttatggcaaggaagctggcatagtatcacaggaataattccagacttaagatcctggttctgctctttagctctgagacctggggaacactaatcagcctctccaaattctctatccagttaagaggagacctaaaaacatccttctcaaatagccccaccacttgagtgcagggtctgtgtattagtccattttcatactgctatgaagaaatacccgagactgggtaatttataaagaaaaagagatttaatggactcacagttccacatggctggggaggccttgcaatcatggcagaaggcaaaggaagagcaaaggtacgtcttacatggcggcaggcaaaagagcgtgtacagaggaactgccctttatcaaaccatcagatcttgtgagacttattcactatcacaagaacagcacaggaaaacccacccttgtgattcagttacctcccaccaggtccctcccacaactcgtaaggattataggagctacagttcaagatgagatttgggtggggacacagccaagccctatcagcctggtaggccctaattcatcctctcattcaacaaaggttttactactacagtgtactgggctgcaagagcacaaagatgaacaaggtagacccagtctctaccatcacggaacctgcagaccaattcgttagctattttcagcagaaacacacaggcatgcctaacatgctccttcgactataaaacacctatcccttctttactttccccactaccagttccactttaacctgtaagtctgggagtagctctggagcatgaattcaggagatccttggcattcgaaggcttaaactctcatggttggcgctattcagaagttctctggtccacagcaagtgctaatttacggtttggccaagacaagatccgaatcctagaggaggcaaggttgttttgtgagggcaagtcctttagctaagaagtaagccaagcctagtgctggcatctcaacttgggtttgttctcttcatttaaccaaaggttttatttaatccttgcaactgctctaataggtaggtatgaccatcctcactgcagtcgcacactgtagtggctgcttagcatttgaaaattcacaagggtcttgtgttatcaccctccaatgctcgtggtctaggcagtggtatctaattctggctatacttagactcaacttggaagctttagaacatactgatgcccaagtcccatctcggatcagtaaaacagtctacctgagagtgaggctcaaatattaggacttttagaaagttatacatattaaggtgcatgcacggtcttccattctggacagttggccccactgggccaaaatccttgcctgatctgcttctagagcccttctaagaagccagcccagtcctctgtggaacatgttcagagcatgttggctagaccaaggaacaaactgccatatggtcaaatgtggatgtgatatggaaactcctgtcacctgactcataaccttccctatccatgcccaaaatgaacttcagaaaatgccaacacaagacttatagtatatgggaatctcaaaatttcgcatgcatttgcaacaaggtctaggagaaacagcatagaaagctgcctaactcttcaacaggagaaaattcatacgatgcattgtataggctttaatgaggacacccaacagttaccctcaaatggaattattctcatgtacccactattttgggatttaattaaaatttcctttaacaactgccaagacattctttaaacttagtctttattaccttctccagaatttttttttttaatactagggtgagcaaaatgttaaatcaggttctcttgatcattatgtatgtattaaacccttggaaacacacagggaaagctaagactcctatcagtttcagtgttcaatacatgaagcatgaaaggcagaatggttcttcaagatgagatgtttaaatggcaacttctttgtcactggatcagaccacacatgtggaacacaagggctgtgtccaagcaggacaactcaatcgcaggctcaggaattagatattgagaaaaagtactaggcgagatcaagagtcaaacagcctgggtagggaagggcaggagtcatccgaacggggtcctcatcccctccagatgtcaaagctccaggggccactgccagccagagctgctgcctctgctctcagctaacagtggctaagaaggaaggcctaggcagctgagtcccaggggagagcacacttggaggggcattaccccaaggaaaaggtggaaaggattataggaaaaaacaaaggttgtctatgtgccacaaggaggggcttcaggttcccgtctctaacataacatttctacagcactaatagcatatcatgtacctgctataccaatagtatagtattaaatacttccatgatagttatgtcttgcaaacagcacccaggtggtcttgactaccaatggactctaaatagagaaacttaacaacctattacatgtgtcagagaacattcactgttgccaagtagtgtttctataggtacgaatgaaggacactcctcttaggcaaaacaggtaaggctttgaggagctgtcacatctacccagctgctttgaggtcattgcttctctgcattttatgttaccccagtctctactcctaggggaggatggttcggcaaggtcaccaagaccctcctggccagagtggggatttctttagaccgcaggagaggagctccttaaccacctttaagcaagttaataatctgttcagggccacctgaggattaagtggtatagcccagagtagagagggtcccccagcatgaaagagactccaatgtcctagtgtcagatgcaaaaaggaaaattacagagctcagcttcctcctaagtgaaaagctgaacttttaaaaccttagacaaatgtgtctatggagtcaaaaacaacacagagaagctgtgacatttaaaaaaaaaaaaaaaaagcaaatgatgaactcaagtaacaaatcttccactcagcatcccagcggcagagagaaatgccaacctcaggactcctacatgtgttttatgctgaaggagctatttcaagcagcaaaggttctgcttctatgccattcccagtttctgttttgttttgttttgaggtatgtctttttaaatatccacgataaaaatgtaaccatcccaaatatatttcaatgatagaaatacatgaccactgtttagtttaaatcaacagtatctctctcaaaactgcctcctggctgggcgcagtggctcatgcctgtaatcccagcactttgggaggccaaggcgggtgcataacttgaggtcaggagttcaagaccagcctggccaacatggtgaaaccccatctctaccaaaaatacaaaaattagccgggtgtggtggcaggtgcctgtaatctcagctactcaggaggctgaggcaggagaattgcttgaacctgggaggcagaggttgcagtgagccgagatcatgccattgcactccagcctcagtgacaagagcaaaaaaaatgccgtctcaacaaaataaaacaaaacaaaactgctttctataaagattactataattgataggaagcccagagcatagtgcctgacacatttgtatgtgctaataaatactagctttcctgattcatataagctaacgattgaaggctactatgaaccaggcactgaaagctctttatacaccttctcaaagactccacacacagcctacaaaggtgctgttatcacatccaatttacagatgagaaaacaggtacacagaggttaaggcaacttcccaaaagtcacactgcaaaaaagagtgcaggctgggattcaactcaaatcaaaggttcttaaacagcagccatgcactttcttaactctaacaacagggtagccctcacgccagaataatttaccatcttttccattttacgctaaagccattttgggggttgtctttaagtgaagtcagagcaggggtggggacactagtcatcaacttgtgcccacccccatcttcggcagcctcccccaggctgtgctcggccctatttgctaaatagcaggtccctggaggttgcacaaccatcagcagcaaagtagctggaatccaaaactaacacggctatcccttcaacgcttcctcttcacctcgggcaaataatccatcagtgcacaaggccacaggtgtgaggggcggcacagagacaggagagaggccccattccaggagagtaagcctttggatctgagcctcacggaacaggcaggctctagcctacagcctccattcctgcagggtaagaatacagtagacaggaggctaaagtggccggtttggctctcgtgatgcagaaggaagcctggagtcagcaaggggagaccaggctgctgaatgggccagtggctaactgcaaggccagctcagggcagctaactgaaacagcagctcctacttcaacgaaggggaactgggtggggagggaaatgacccagtgtagacattgtccttacagcacacacaaaaagcacatgcctacatatgacaatgatggaatatggcatttcaagccaaatttatactaaacatcaaagaaaaccagggcttttctgaaaccaaaacacatttctaaccactttcttgaagaaaacaaaaatggctgggatctgaaccaggcataaccattttgtcttgctttttgaaagctgacaaatggtcatcccagcccttccttccccagtctatgaccttttcagaccatcttggttcctctcctgatgtttcctaaagtagtgaaatgacagtacattcaactatctggccccattttatttccatgtgatttaaacctgatgtttaatgtgacagcacttccatttaaagtaagcaaaaaaaaaagaaaaaaagtttcttatacacaaatgttttaacgtttaatgtgtaatgtttaacatgtggttaaaaaggaagcagcccacaattttaaaaaaatgaaatttaaaaaatggaagaaaaacaatgaccccaaaatcctcattcaaggaattgtgaacagaaacaaagtcttacaatagcctgcagtacactatcaaatactagctttatgtatatatagatatatacgtatatacacatatagatatgtacacatatatacagatatatgtacatgcaaggatccaaacctagtagggaatttccaagagtgccagcttctctgacaccctggaaaggaactcagaaacacaggtgtctctccagactagaaaacctcaactggaggccagaggtgggacacgccctaggaagcatccagacagacggagtggaacaacacaacctttccaacacgaaggagcccactgccatatctgaatctggctgcaaatctgtcaagacacagggcgggtggaaacatcagaaaccatcttactgacatggtcaaccaatggctgagcagacacactcaggaccaagaccccataatacagcagttaaaagcctccaggctctggaatcagagcccagttgcagcctcttccagtgtcaataagagaagttaccaagtggatggtggtgaggccataacaagccggtacccacatgcggtgggggctctgacaccactcccatttccattatcaaaccaaggagaccgaaaaagtgacctgggccataggattctcaaatactgatcatctgaacaaatagaatcttgtatctgacaacagcagagcagcacaaccatttggtttgcagccacggccaaaacttggagattgcaaatgtacaatcagagtaaagacagccacaggatagcaaaaacctttctttatttctttttttctagacgaatgaactgtaagctactttgcattccttttaagcttcttattttttagtgtctgataccacggccattaaaaacaatctctaaaaagtctttgttgcacatcagaatgagacagctgggttactggcatgaggaaatgttcaatcttgtcattttgcaaaggaattcatattcataattaatgacgcttttgtccatgccagaaggaaaatctaaaggctcaactatgcctaagtaaattctaaccaagccaactgcaacacggttttataaattatagagcaacagaaaagaacaagattttgtgagttgcaagcataaagaaaagaacgaatgacaaggcggccatgtttcaaggaagcaatgagattaggaacattcatttctaaaaggatgggtagattttccttctccctcataaaagcagcagtaattgaaaacttcaacatcataagaaaaggcatatatttgacctgctacatgtatttgagagatttaataacactttctttgtgagtgtgccagacagataccaccgggttccatcactggccccaaatgtcaactaaagataatgaagtgggggcagataagctacaaagttaggtttggtttaagaggtatgtctatggagatgctggtagataagtagaaaaccccttgaaaaaacactagtgaaacatttcaaagaaatgttcttaaagataactttgcttgtcacatagccattagatagataaacaaatgtgtgttcaagtagaaactcattccattcattcaaagaagatgtatttggcccctactatgttaggggctaaggctataatgataaaacacaaaacactgccagaagctgggaagggtggggacagggagtaactgcttaatgagtatgagatttttgtgtgtttttctcatggtaaataaataaataaatataaaccaagaaattcactattttaatta

SEQ ID NO: 13938 - RNA, 848 nt, Homo sapiens
  source 1..848: mol_type = other RNA
gctgggattacaggcatgagccaccatgtctggcccagaaagcattttgataaaactctggttcccagcactcaaacctggtgcctcaaacacagtaggtgcactgcaaatgtgtgctaagtgaaggtaagacatgcttactttaaataattcacaagacagaagaccgcacttaaaaaaatctacaaggaaacaccaatttaaagaaaagaaaaatcagtaagtatctgtgagaataatggagcaaaagaagtcctgaaagagttctgcatcttggtggtcatatttattggagagcttgagaaaaatgaaaataccatttagcttaagaagttgtgagttatctgcaaatcaactcatttcaggagtggaagaatccccggaattatttcttaatatcaaaatgtatgcaggtttctcttatgaatgttttgtacttttagagaggccactgtacaaagtctcccgttttccatacaggacaaattctttgtttcagccaactctcagtggaggggcaaccaggacaacgccatctccccggacaaagagcattggaatattccgtttcgttgatttatatatctcttcatatgtttcttcatcaatttctatagtagtcacagtttcttccacatctcccaagatcatatttaaatgttgatcataagcatgtaatctgcctcgaagctctcggtcatttctcattttcacataaattcgctcatctaggctgagcctgataagatccaggggctcctctacagtgttggtagtttgttgctggtctacgtcgtccgccatgtttcaaaccctgcgccctttcccgcctctcgcgagaacacaag

SEQ ID NO: 13939 - RNA, 90 nt, Homo sapiens
  source 1..90: mol_type = other RNA
gctgggattacaggcatgagccaccatgtctggccctactcgcctgcgcttcacctcacgtgaggattttccaggttcctcccagtctct

SEQ ID NO: 13940 - RNA, 2220 nt, Homo sapiens
  source 1..2220: mol_type = other RNA
gctgggattacaggcatgagccaccatgtctggcctggttctttcaactggtgttttacctcttcctcagatgtccatcactatccctgttgctctcctctttatcctctccggcctggctctgtccctcttatagcaaggggcctggaactcaacctagcgcgaatggtctaagggttctgtcctggtgtgggacacttcccttctgttgatgcagccctgtggtgggcttttctggaagcctcaccacactggtgttcaacctgagcttactgtcaggtgaagcccctaaattgatgctttctgatcctaactctctattctatttttatataatggggattctgtgcccaggtacaggaatttacattcatccctattaaatattttcacctacatgcttcttggttctgtctgttacatcccctatggacacacacacacacacacacacacacacacacactcctctttcccagaagacagatgtgtattttggacaatctactccatggggactatctgttttccactcttacccttaaaagtaaggaaacacaagttgtgtacatgtttcctccagggttttcctggtcacattgcatactcaggcgagagggcttcatgaccaagcgtgcaggctctgggtcagactgcctgggttggaatcccagcctgagcacggagccttgtgaccttgagatattaatgtagcctctgtacttcagtgttctctgtaaaatagcgataactatatctatctcacttgttattctgagaattaaatgtgatagttggccgggtgcagtggctcacacctgtaatcccagcactttgggaggctgagcaggtgagtggcttaaggccaggagttcgagaccggcctggccaacatggtgaaaccccatctctactaaaaataaaaaaatagccaggtgtggtggcatgtgcctgtaatcccagctactcaggaggctgaggtatgagcatcgcttgaacctgggaggcggagtttgcagtgagccgagatcacaccacttcactccagtctgggagacagagtgagaccctgtctcacacacacaccaaaaaatgtgatagtaattgggcagtaaatatgttggcctcctcgttgcctcttctggcttctctgggtcccccgatcttgctttcccatcctgacaccctcccacatctgtttgaccttagttacaaagagaaacacagaatttctgtgatgaaagggcttcagaggcagtccaatccagcccctttgttgtacagatgagaaaaccacagtccctcctgccattcctctgttgcttcattttgttccaaagtcgttgtatttccagcactccagttaccaccttttctctctccagctcacatagcaatcagatcaggctgcttttccccagtgcaatcagtgagctcccagcctccagcttgctggatttatggctctctgctggctcacggggtccttaggggtctgtgtagctcaggagttatgggccagccgagacagggctttcagtgcacttggcccaacttgtcagtcacctcctggggccggttgcatggaaaaaagaaaatcaaataccaaggccaatatgctgaccacatttttatgctcttcattcaaatccaaaatgttccctatggggcatgctggaagctgttcagaactgaaaggcagagatcgttctccaactggccaggaaaggaggactacagggaggatgccgcatgtctgagcagtttgtgtcccttctcagaagacgttgtgcccatgtgccagggcagtgcaatgacagagggtggtggggtagaagctctgatttctctgaattctccattaattccttggccgcgcggcctccggcggcggcgccgcagcttttgtctcccgcccgccgggctgcgaggtgcgggcgcttaggcgcgaagttgcagctccgacgcgctgctccggaatgccggctgaccgcggccgtcggggggcgcggagggcggggtgggccgggcacgccggccccggggctggggggcttaatgcatatttatgccgcgccgaaataggcttcataattaactcccggagtcatccgcagaggttaaagggaccccgaagatttgtgcattgattgggtacctcggcggggtgtgtgtgcgcgcgcgtgtgtgcgtgcgccccgtgctaacccattgaagaat

SEQ ID NO: 13941 - RNA, 1511 nt, Homo sapiens
  source 1..1511: mol_type = other RNA
gctgggattacaggcatgagccacccaccatacctggcccaccaattgttaatattttgccacatttgtgttctctctttcatatacaggcacagacacatatatacatatttttttttctgaactatttgaaagttagttgcaaacatgacacttttatctctaaatactgtacttcagcatatgtcttctgagtacaaggacattcccccatataaccacaataatcaaacccaggaaatttaactattacctaagactattatctaactatagtccatattcaaatttccccaagtatctagtaatgtcctctatacctgttaacttattgaggatcttgcattgcatttgtctcttttagtctagatttaagtacctttgttttgtcattatgacattgactattttgaagagttgaagtcaggttccatcctcccatccctatcgcaatgtccttcaatttgtatctgtctgattctttctttctatttttttgagacagggtctcactctgttgtccaggctggaatgcagcagtgcaatcttggctcactgcaacttcggcctcctggtctcaagcgatcctcccacctcagtctctcaagtagctaggactatagtcacatgccaccatgcccagctaatttttgtattttttgtagagatggagttttgccatgttgcccaggttggtcttgaactcctaggctcaagtagtctacatgtctcagccttccaaagtgctgggattacaggcatgagccactgtgcccagcctgattgtttctttatgatgagactcaggttaaatatttttggcagaatattacaaataagtcatgtttcaatgccaccttttataaatgtttcttatccttctcttttaaatgtgtgaagccaggaataataaaaagtctaataatcttattttcaaatatctagcaggtcatttattggcaagtgactcttgtcatcacgtcatgattgaggcagtaggctatttatacagatcagttgatttaagggtgatccacctgggatcttctcattcatcaatccatggaatccatggaatcctgcagtgagtttctgtttcatgttccaaacagaaatatgcttctggttattcatgctatatatatgacctcttgacaacttttgatcttttgcagccttctgagagaaattgagtggatccggagccggagatattggcctcaaggtatgagccagcaacattctgagggttctaggaatggcttctcattatgggagcacttggttaaattaaactaccacagtgctcagagttctaatacagtgagctctgcaatgtgcatgaatgcagataaattacacagggctagaagaatggacttggcacctcagacaatttcagataaatcaaaatgtgctcctcatcattccatcccatgtggcctgcgcgccaccacaccacacggccacccccgcgccaccctgaaattgaccgcagcaggctgggcgtg

SEQ ID NO: 13942 - RNA, 3334 nt, Homo sapiens
  source 1..3334: mol_type = other RNA
gctgggattacaggcatgagccacccagcgcccagcctcacagattgatttctttttttttctttttgagacacagtctctctcagttgcccaggctgagtgcagtggcgcgatcttggctcactgcaagctccgcctcctgggttcatgccattctcctgcctcagcctcccaagtagttgggactacagatgcccgccactgcgcccggctaatttttttgtatttttagtagagacggggtttcaccgtgttaagtcaggatggtctcaatctcctgacctcatgatccgcccatctcggcctcccaaggtgttgggattacaggcgtgagccaccacacccggccacagattgatttcttatgagtcaggctgtgtgatgaagaagcccagaagagaaagaagcggaaagaaaaggaatcaggaaagactcttactcagcgtcacttgacattcatggatgtggctacagaattctctcaggaggagtggaaataactggaccctgcacagagggctttatacagggaagtgatgtaggagaactacaggaacctggtctttctgggaatctgtcttcctgacctgagcattatctccatgttggagacaaagcgagagctctggactctgcagggtgaagatagcaaacaatccagatggcagggaatgcatcaaaggtgtgaacacagggagaagctctctatcaaattcatcctcctcctccaaaagatcatacacctgctctaaaagctgaactcccaggccacgaattacatcagttctcaagacttcaactagtctcctgatcttttcagaacctggcataatagctgaaggtagctctttaaaatggatttcctctgcctcttctgcaaccttcccatgaagtatcagtgtgtcccgatatttccgatgaagtttgaattctgacactgggtttgctaccgggacatcttcacagctctctttagaatccagtttcagggtctgagtcatcaattgtaccaaggcattaatttcatttgtctgacctttcccttccccgtaatccccatctgacttatcagttgaacttgtagaagaacttaactcatcctcagacagacaatgaatctgtttcctttcctgagtgacgctgcagtcagaggagagccgtcgggcaggcaagggctggtcttcttcctggggttttcctggccctgctacactcagagacgctttcctcactgaagggcctgaagaggacatttcttcctgtgactgctttagtcgcctcctctctctggctgataatggtcgatcctttgatgatgacatctcactgctccttgaactgctcacagacccagtgaccactctacgttggttttcagcctctttttgtgttgatgtgacatccactttcccaacaatgggatgagaaggcaaaaatcgaggaggcgactcttggaaagcaaagagatctctgcggacctgtctcttttcccctctgtgctcagtctgttctctcctcttttgccgtcgctgtcgagacagggaaggttcagacccagagttgtgtggctgtaaatctgggtggattctgccctgtttttctataatacattcaccagcaacttgatcctgggcgtggtggcacacgcctgtaatcccagctactcgggaggctgaggctggagaatcacttgaacccaggaggcggaggttgctgtgagccaagattgtgccactgcactccagcttgggcgacagggcaagactctggtcctttggcttttgttctttgattaggggctgcagaggcttcactggttcattcttttccccagtgacaatgtcagaggaccacatgggaatcaggttttcaggctgggcactggatttagtgttgtcctgcagcatctcctcttccacttgagaaatactgcatatacctcctaactcattagaggcatccaaatatcttggctgattctcctgaacaaagccatcactcactgaatccctcccttttgcaggtaagatgtcaatatttacgctactgattgtggctagttctgtggtattgctcaagtcctgtttgcaggtatgggctttcagactggcaggtgacttcaagagaccagaggccctgggtttctcctgggacaaacatttgccttcacccattatatatgtctgggagccctcagaagagagtggttgggggtggattacttcatgatttgattctgcctctccagaaaccactgtagcaaaaggcttggattgagagtcaccatttttaatgttatttttggaggtttttatctttgtggcctccaaaaagaaggagatttgccgctttatataaggctgcctcaggatgctcctcacagacggcctttcttcaggccttttgctcagcattgttcttatcagttctgccagctctgggctgtaatctcttggcattggtggcagctttccttcaataatccgataaactaaagaattcatatcttttgcattgaaagcatgcttcaaggtggccatttcatagacacagcatcctagagcccaaacatcagacttatagttgtagggtttgtttgagaacaattcagggctcatgtagtagggtgtgccaatgagggtgctagccatgtcacagtggttctctaacactcgggcaattcctaggtcccctactttgatgatgtttgttcttgttaggaagacattttgagttttcagatctcgatgaaggatgtgtttttcatgtaaatactgcaaagccatggcgatctgtacaaaccactctaccacctgattctcaggcagaagctgccctttctgctccttgagctttcggtacaaatcacctccttcacagaagcccatgacaatgtagagcagaccatctcctccttcccatgactccttgtaggtgacaatgttgggatgcttcaactgagacaagagctgggcttcctgttcagcagctcgccgctctcggctagaggcatttcggaggttcagttttttgatgacatactgcttgccgtcccgccggtgcttcacaagcgtcacctctccatagctccccttgcccacgacccgcaggtagcagtaggcggccaggggcatgttcccagcgctggcccagagtcgggatgcggcggcagcggcgggtagggcagcgggcggcaacaagaagctcggttcatgcccgagagggggcagtgggggcggctgttgaggcagccgggcccgggcgggattgctggggcccggcccgcgacgacgccgctgccatagcgatccgggccgggagcagttctgcgcat

SEQ ID NO: 13943 - RNA, 3196 nt, Homo sapiens
  source 1..3196: mol_type = other RNA
gctgggattacaggcatgagccacccagcgcccagcctcacagattgatttctttttttttctttttgagacacagtctctctcagttgcccaggctgagtgcagtggcgcgatcttggctcactgcaagctccgcctcctgggttcatgccattctcctgcctcagcctcccaagtagttgggactacagatgcccgccactgcgcccggctaatttttttgtatttttagtagagacggggtttcaccgtgttaagtcaggatggtctcaatctcctgacctcatgatccgcccatctcggcctcccaaggtgttgggattacaggcgtgagccaccacacccggccacagattgatttcttatgagtcaggctgtgtgatgaagaagcccagaagagaaagaagcggaaagaaaaggaatcaggaaagactcttactcagcgtcacttgacattcatggatgtggctacagaattctctcaggaggagtggaaataactggaccctgcacagagggctttatacagggaagtgatgtaggagaactacaggaacctggtctttctgggaatctgtcttcctgacctgagcattatctccatgttggagacaaagcgagagctctggactctgcagggtgaagatagcaaacaatccagatggcagggaatgcatcaaaggtgtgaacacagggagaagctctctatcaaattcatcctcctcctccaaaagatcatacacctgctctaaaagctgaactcccaggccacgaattacatcagttctcaagacttcaactagtctcctgatcttttcagaacctggcataatagctgaaggtagctctttaaaatggatttcctctgcctcttctgcaaccttcccatgaagtatcagtgtgtcccgatatttccgatgaagtttgaattctgacactgggtttgctaccgggacatcttcacagctctctttagaatccagtttcagggtctgagtcatcaattgtaccaaggcattaatttcatttgtctgacctttcccttccccgtaatccccatctgacttatcagttgaacttgtagaagaacttaactcatcctcagacagacaatgaatctgtttcctttcctgagtgacgctgcagtcagaggagagccgtcgggcaggcaagggctggtcttcttcctggggttttcctggccctgctacactcagagacgctttcctcactgaagggcctgaagaggacatttcttcctgtgactgctttagtcgcctcctctctctggctgataatggtcgatcctttgatgatgacatctcactgctccttgaactgctcacagacccagtgaccactctacgttggttttcagcctctttttgtgttgatgtgacatccactttcccaacaatgggatgagaaggcaaaaatcgaggaggcgactcttggaaagcaaagagatctctgcggacctgtctcttttcccctctgtgctcagtctgttctctcctcttttgccgtcgctgtcgagacagggaaggttcagacccagagttgtgtggctgtaaatctgggtggattctgccctgtttttctataatacattcaccagcaacttgatcctggtcctttggcttttgttctttgattaggggctgcagaggcttcactggttcattcttttccccagtgacaatgtcagaggaccacatgggaatcaggttttcaggctgggcactggatttagtgttgtcctgcagcatctcctcttccacttgagaaatactgcatatacctcctaactcattagaggcatccaaatatcttggctgattctcctgaacaaagccatcactcactgaatccctcccttttgcaggtaagatgtcaatatttacgctactgattgtggctagttctgtggtattgctcaagtcctgtttgcaggtatgggctttcagactggcaggtgacttcaagagaccagaggccctgggtttctcctgggacaaacatttgccttcacccattatatatgtctgggagccctcagaagagagtggttgggggtggattacttcatgatttgattctgcctctccagaaaccactgtagcaaaaggcttggattgagagtcaccatttttaatgttatttttggaggtttttatctttgtggcctccaaaaagaaggagatttgccgctttatataaggctgcctcaggatgctcctcacagacggcctttcttcaggccttttgctcagcattgttcttatcagttctgccagctctgggctgtaatctcttggcattggtggcagctttccttcaataatccgataaactaaagaattcatatcttttgcattgaaagcatgcttcaaggtggccatttcatagacacagcatcctagagcccaaacatcagacttatagttgtagggtttgtttgagaacaattcagggctcatgtagtagggtgtgccaatgagggtgctagccatgtcacagtggttctctaacactcgggcaattcctaggtcccctactttgatgatgtttgttcttgttaggaagacattttgagttttcagatctcgatgaaggatgtgtttttcatgtaaatactgcaaagccatggcgatctgtacaaaccactctaccacctgattctcaggcagaagctgccctttctgctccttgagctttcggtacaaatcacctccttcacagaagcccatgacaatgtagagcagaccatctcctccttcccatgactccttgtaggtgacaatgttgggatgcttcaactgagacaagagctgggcttcctgttcagcagctcgccgctctcggctagaggcatttcggaggttcagttttttgatgacatactgcttgccgtcccgccggtgcttcacaagcgtcacctctccatagctccccttgcccacgacccgcaggtagcagtaggcggccaggggcatgttcccagcgctggcccagagtcgggatgcggcggcagcggcgggtagggcagcgggcggcaacaagaagctcggttcatgcccgagagggggcagtgggggcggctgttgaggcagccgggcccgggcgggattgctggggcccggcccgcgacgacgccgctgccatagcgatccgggccgggagcagttctgcgcat

SEQ ID NO: 13944 - RNA, 6340 nt, Homo sapiens
  source 1..6340: mol_type = other RNA
gctgggattacaggcatgagccaccccaccccaccccaaagtgattttaacttcagcaatagttaaaactgtttctatccaggttaaacaggatttaatcttccatctaattactatcaaaaatataggcaaccttccccaaaagtgggcttctgaaaataaatacttggttcagtaaatcaataatttctggtaaacatccttaatttacttaaaaaaatcctaagacacactgtatgcacactgtaccttacaaatctgggacactggccacatttcaaaatactacacttaggaatttctgtaattggccaagtcacatgatttattaaaggaatagttgaacagattccctatattattttcctcttacagggaattaaaataagctactaggttcaagtagaaactgtggagagaagacgaatccaatgttttcaaacaagtcacataaacagaaactaaaaacctaattgcaagccaacacatatgcataatcaaaaaccaaaactggttaagggttttaggtaatctgtaatcatctttttactcatttaggccttgatttgagacatgaaagcatgaacaaggcagtttaatttcagtgttgtactgaggtgatatctatccactaataagaatgtaaatataaacaagttttatctcacatgtgccaccatctctcctttactatagtctgttaagagttgacaggcccacctatggtccccagaatctcaacattaaacaaatataaatcccaaaaggcattactaccttagaaccagaaattcttagttatcatcttgtgccacacggccattacttgatcagcaactttaacttaacccctcatcccacataagacattgctaatttttttttggtacattaggcagttagctaaaacctgatattcaaataaatgctgatgttacttcaagtttaaaaactgctgaactaaaaaggtcaacaattatctatatgcagcattgcaaagattcctttaagtagcacaaaaagaaaactgcaatataaaaaacatctttatagatttgacaaatgcaaccatttaaaagaaatgtcactcagcataaacagtggtctacaaatctaagctcttcaaaaaggttacctgtaagttctaaaatggccttctataaagtgcaacattttccattaaatcgttaaattctacaagggtttttcaaatagagggatgaagaaaagtatcagaaggtgacagtttataagcacaaaacacaaattctataaactcacctggattatactataataaaaatattattattcacatccagatttgaagtttgcattaaattatcaaacctgatgagaaaaaacttaaaaacaaaccaccattattgtgttaccatatataatctgcaaatcaaaaaaagactcacaaaacccaagtttaattatcttgtttgccctaaaggaaattaagaactgtaatgttaaccttgttctgaatgtattccagactcaagtctccctacagtaggaagttcattgcggtctatgctactgaaatgtaattaggggggcattatggttctagagaaaaagcatcagtttgggaggcaaatgtgctccttgctacatggatgacttggaagcctgtcatttaactgttctgattcagtttcttcctcatctattgtgctgaggacaatatcacctaacccgcagcacagatgtgaaaattaacttttctaacctaaagtgcaattcaactaacactgtggtaatgacatactcaaccaaagtcaaattattatttttggattatctatctcactggtccctagcaatatctgacaaagttgagaacgctggaatacacaaagtaaaacccaacctcaccactaaaacaaaaatacagtttaaggcccaagatgtctaattacaaattaacaggtcttaaaaaactaagacccactgaaccaaacaaatcttatctaactaaaatactcatgaggccaggtgcaatggtgcacacctgtagttccggctacttggaaggcaggagaactgatgaggccaggagcttgagaccagcctgacaacatagcaagaccttgcctctataaaaataaaaatttaaaaaaaaaatctcatgggtcaagagttctaagctcagtagctaataactatacattgggccattcctacggatgaaaattttcattttaaaatctgaaaatgttcaatgtgatgagctcctactgctgccacctatagaaaatgttgccctaacttataatgattttccagcagtggaaacgtatacatctctaagctctcaggtttactctacatgcaataatgtacataattgtacaaggattctcaacagttctgatcatgatgctaatcctatttcttaggtccaatactatcattcaaaacctcacaatcatcccaactctgatgacagaaagcactggggaagctttctattttctgagattgtgcagtaattccctgcaacaaattacaagcagcatcagtatgtattgctaccacctctccacatttacaccaacatacacaacacacacatacatttggtacaaataataaaaagtgaaattactaattccttagagtagatgttactgcaattcttgaaacagatttccatttcctagtttgttatttatctgaggctgagtttcaaaagaatgagtcttcattccagttttcctaatcccacagctccacccacccacaggaatagggactatcagtgttctcaatggggttgcttcatttttacacaacatttggtatccttagaccccacccaataaatgccagatgcatgtctctccaacaacccttccaaatttcacacatttccaaatgtcctctagtatgtgataacaccaagctgaggattgctgcatctagttaatgcccttaagtctccaagtaggaagaacttctgttttgaaatgtataatttagtattcactcatgaaggataatttctaggctatccataatttatgaccttgaagttaccacaaagtaatttttttttccaaagtgactcagactaaacttttctttccacccaccacatgcttaatataagctacaaaagtataagttgtatttcttcctattatcagtgatctgggccaaaagtggttaccaaagttactttaaccctacaaaaaagccatgtgattcagttacattaagtttatgtaaaggagatgctgccaattttcaaatatttgaggaactggaaccaaactggtaataccaacttcactgtggtcttaaccatcacagcaaacctagagtttctcagtaatgcaaaccaaatattcctatgctatcctcaaacgacagtcctaaagatgaatactgttaagaaaataaatacgctgaattttacaacctggttgcccttcaattagtaatgacaatcacacaaaagtttgtttcacacgtgtaaacaaaaccttcacccatctcacacacagcactcaacaaataacacatatgtgaaacgagtattagtctatattgccagattaaattttcttccagaaatattttaataaaaattggccatttccaagtaacacccactgcatgcccatcaataaaagagaaccataacaaaatagaaaatttaccatatggctatgattttaagaaaaaaaaaaatgcggacacgagcacatgagcaaagtccaatattaaagtaacattccttcttacgggctatgattaggaatctgattagataccagaataaaaatacaaatgctgaactatttaggtcaaagaacctctatagaagcatctgtcttcaaaggcattccagtttgagactcaattttagaataaggcataacaaatatgttaacaaaagacatacacaaagtgatgaaagagggattctataattccccacatactctgaacctaataaaacaaatctagattttttttttaaacaattgccaagactgaaatcaaagataaatagaaggcacaacagttttgctctggttgttatctgggttttgggaatttttttgctttttgtttttttacaaatacaaattaaacatgaaaaaactacttcaaaaaaactaacagttcaagaaaagcctatcagttgcattctagacatttaaaacctattatcacaatttaaatttcaatggtaaaaacagttaggttttagaattgttttgtgatcctttatcaaaaaaaaattctattccttttattcagtttttaaacataccagtgagaatcaaaattgtcaaattttccaatggcaatttctccacaccagaaggtagtcatgactctcaaagaagaaacaatttgggtttttcctgccttcaaaatattatcaaatcctgtatttcttacaggcttttcaaacacgtagaaaataagaaatattccaatgaatgaaacataccaaatgtcagtaatatgcaagacattcctttggggaaatggctgtaaaaaaaaaaaaaaaatccagtctgtatatgcaaagtaagcaaggaaattcagtctttttttttgcttctttaaaagtccgttattcctaaaatatcattccacaaaattggaagtgaaagactaaaggtcaggaaagggaagagagggagagggagcacacaccattaacacacaaaaaaagtaaaattatacaaacttaagcagtttataacagactggggtcatactccaagataccaaaggctgtcgaaaattcaccattctgttggaaccagggtttgtatggctgcatgaagatccatgaagattcactgccgtggcgcaagcccccttcccactccaaatcctggtttctgcaccatgcctccacggggagggcctctcattccaccacccagcccacctcgagggcctccaggtccccgaaggcgattatctcgtcggtcgccttccctggcagctcgagtcttcttctcttcgacattcagacggacctcacctctgaacatgatgggcctgttgctaaggactttctgaacaggctcagaatcatcaaacacaacaaaaccaaaattgggtaatttcccaccactgttaatgcgcaactccaccacgtttccataactttgaaagaaatctttaagctctgatttgtccacttcatgaggcaggttgccaatgaagagttggtgactgtcagggtgtctcaccattcttcggggttcaatgtcaccttgctcaccagcctcacggattggtctgggtcccctttggggaggaatatttattcgttgttctcgcactctttgatcccgctgaggtctttgtggtggaatctgagattcaggcttagactctggacggggctgtgaagctggtactttaacaacatgaggtggtatcccagtaactggaacagctccactgggtggaagattcttactggtcacagatgcccaagaaaatgtcctcaagtcttcctgtactgtctgagctatgtctgcaggtgctggagaagaactcttctgagcatcctcaggggcagtttcttctaatactggctcaggcttttcctcttggatttcagatacaggttcttgttctggttctggttcaggatcaggctctggttcagcaacaggctcctctaaatgttcttccatgtcattactgacaactgcctgatcatagaaagttccagaatcatcaggtaccacctcaggtgtttgctgtctttcttcaggttcctctacttcttcttcagactcctcctgaggctcagtgacaaacccaccaaagacctcatcttggtatctgaagatatcattgtgaacatagaatttatttgcaacagacccctcaggagcaaggacaaacgtttgcatgaatctcctcaaagcctggttgttgttagagagaagccccatcacctggactaccacaccatcatttagcgtggcatgagcatcaacatggcgaatcttggtgtggcagttggtgaagttttgtgacatcactttcctgtggatttctttctgtccgtagactgcatctgctggctttccatttgaatccaatcccccatggacataagaagagttctttccataaaatctatgcagcatgtctggggcctggttcagcagtgtgtaatactgtctcacaaattcccgcccgaccagcaggggactaggcttctccatcaccattgctttggtcaattcaacctacgcggctgagctggagaggaactagctctgcaccacagcaccgaggatagtacaaacccctcacgcaactgcgtccgcac

SEQ ID NO: 13945 - RNA, 6371 nt, Homo sapiens
  source 1..6371: mol_type = other RNA
gctgggattacaggcatgagccaccccaccccaccccaaagtgattttaacttcagcaatagttaaaactgtttctatccaggttaaacaggatttaatcttccatctaattactatcaaaaatataggcaaccttccccaaaagtgggcttctgaaaataaatacttggttcagtaaatcaataatttctggtaaacatccttaatttacttaaaaaaatcctaagacacactgtatgcacactgtaccttacaaatctgggacactggccacatttcaaaatactacacttaggaatttctgtaattggccaagtcacatgatttattaaaggaatagttgaacagattccctatattattttcctcttacagggaattaaaataagctactaggttcaagtagaaactgtggagagaagacgaatccaatgttttcaaacaagtcacataaacagaaactaaaaacctaattgcaagccaacacatatgcataatcaaaaaccaaaactggttaagggttttaggtaatctgtaatcatctttttactcatttaggccttgatttgagacatgaaagcatgaacaaggcagtttaatttcagtgttgtactgaggtgatatctatccactaataagaatgtaaatataaacaagttttatctcacatgtgccaccatctctcctttactatagtctgttaagagttgacaggcccacctatggtccccagaatctcaacattaaacaaatataaatcccaaaaggcattactaccttagaaccagaaattcttagttatcatcttgtgccacacggccattacttgatcagcaactttaacttaacccctcatcccacataagacattgctaatttttttttggtacattaggcagttagctaaaacctgatattcaaataaatgctgatgttacttcaagtttaaaaactgctgaactaaaaaggtcaacaattatctatatgcagcattgcaaagattcctttaagtagcacaaaaagaaaactgcaatataaaaaacatctttatagatttgacaaatgcaaccatttaaaagaaatgtcactcagcataaacagtggtctacaaatctaagctcttcaaaaaggttacctgtaagttctaaaatggccttctataaagtgcaacattttccattaaatcgttaaattctacaagggtttttcaaatagagggatgaagaaaagtatcagaaggtgacagtttataagcacaaaacacaaattctataaactcacctggattatactataataaaaatattattattcacatccagatttgaagtttgcattaaattatcaaacctgatgagaaaaaacttaaaaacaaaccaccattattgtgttaccatatataatctgcaaatcaaaaaaagactcacaaaacccaagtttaattatcttgtttgccctaaaggaaattaagaactgtaatgttaaccttgttctgaatgtattccagactcaagtctccctacagtaggaagttcattgcggtctatgctactgaaatgtaattaggggggcattatggttctagagaaaaagcatcagtttgggaggcaaatgtgctccttgctacatggatgacttggaagcctgtcatttaactgttctgattcagtttcttcctcatctattgtgctgaggacaatatcacctaacccgcagcacagatgtgaaaattaacttttctaacctaaagtgcaattcaactaacactgtggtaatgacatactcaaccaaagtcaaattattatttttggattatctatctcactggtccctagcaatatctgacaaagttgagaacgctggaatacacaaagtaaaacccaacctcaccactaaaacaaaaatacagtttaaggcccaagatgtctaattacaaattaacaggtcttaaaaaactaagacccactgaaccaaacaaatcttatctaactaaaatactcatgaggccaggtgcaatggtgcacacctgtagttccggctacttggaaggcaggagaactgatgaggccaggagcttgagaccagcctgacaacatagcaagaccttgcctctataaaaataaaaatttaaaaaaaaaatctcatgggtcaagagttctaagctcagtagctaataactatacattgggccattcctacggatgaaaattttcattttaaaatctgaaaatgttcaatgtgatgagctcctactgctgccacctatagaaaatgttgccctaacttataatgattttccagcagtggaaacgtatacatctctaagctctcaggtttactctacatgcaataatgtacataattgtacaaggattctcaacagttctgatcatgatgctaatcctatttcttaggtccaatactatcattcaaaacctcacaatcatcccaactctgatgacagaaagcactggggaagctttctattttctgagattgtgcagtaattccctgcaacaaattacaagcagcatcagtatgtattgctaccacctctccacatttacaccaacatacacaacacacacatacatttggtacaaataataaaaagtgaaattactaattccttagagtagatgttactgcaattcttgaaacagatttccatttcctagtttgttatttatctgaggctgagtttcaaaagaatgagtcttcattccagttttcctaatcccacagctccacccacccacaggaatagggactatcagtgttctcaatggggttgcttcatttttacacaacatttggtatccttagaccccacccaataaatgccagatgcatgtctctccaacaacccttccaaatttcacacatttccaaatgtcctctagtatgtgataacaccaagctgaggattgctgcatctagttaatgcccttaagtctccaagtaggaagaacttctgttttgaaatgtataatttagtattcactcatgaaggataatttctaggctatccataatttatgaccttgaagttaccacaaagtaatttttttttccaaagtgactcagactaaacttttctttccacccaccacatgcttaatataagctacaaaagtataagttgtatttcttcctattatcagtgatctgggccaaaagtggttaccaaagttactttaaccctacaaaaaagccatgtgattcagttacattaagtttatgtaaaggagatgctgccaattttcaaatatttgaggaactggaaccaaactggtaataccaacttcactgtggtcttaaccatcacagcaaacctagagtttctcagtaatgcaaaccaaatattcctatgctatcctcaaacgacagtcctaaagatgaatactgttaagaaaataaatacgctgaattttacaacctggttgcccttcaattagtaatgacaatcacacaaaagtttgtttcacacgtgtaaacaaaaccttcacccatctcacacacagcactcaacaaataacacatatgtgaaacgagtattagtctatattgccagattaaattttcttccagaaatattttaataaaaattggccatttccaagtaacacccactgcatgcccatcaataaaagagaaccataacaaaatagaaaatttaccatatggctatgattttaagaaaaaaaaaaatgcggacacgagcacatgagcaaagtccaatattaaagtaacattccttcttacgggctatgattaggaatctgattagataccagaataaaaatacaaatgctgaactatttaggtcaaagaacctctatagaagcatctgtcttcaaaggcattccagtttgagactcaattttagaataaggcataacaaatatgttaacaaaagacatacacaaagtgatgaaagagggattctataattccccacatactctgaacctaataaaacaaatctagattttttttttaaacaattgccaagactgaaatcaaagataaatagaaggcacaacagttttgctctggttgttatctgggttttgggaatttttttgctttttgtttttttacaaatacaaattaaacatgaaaaaactacttcaaaaaaactaacagttcaagaaaagcctatcagttgcattctagacatttaaaacctattatcacaatttaaatttcaatggtaaaaacagttaggttttagaattgttttgtgatcctttatcaaaaaaaaattctattccttttattcagtttttaaacataccagtgagaatcaaaattgtcaaattttccaatggcaatttctccacaccagaaggtagtcatgactctcaaagaagaaacaatttgggtttttcctgccttcaaaatattatcaaatcctgtatttcttacaggcttttcaaacacgtagaaaataagaaatattccaatgaatgaaacataccaaatgtcagtaatatgcaagacattcctttggggaaatggctgtaaaaaaaaaaaaaaaatccagtctgtatatgcaaagtaagcaaggaaattcagtctttttttttgcttctttaaaagtccgttattcctaaaatatcattccacaaaattggaagtgaaagactaaaggtcaggaaagggaagagagggagagggagcacacaccattaacacacaaaaaaagtaaaattatacaaacttaagcagtttataacagactggggtcatactccaagataccaaaggctgtcgaaaattcaccattctgttggaaccagggtttgtatggctgcatgaagatccatgaagattcactgccgtggcgcaagcccccttcccactccaaatcctggtttctgcaccatgcctccacggggagggcctctcattccaccacccagcccacctcgagggcctccaggtccccgaaggcgattatctcgtcggtcgccttccctggcagctcgagtcttcttctcttcgacattcagacggacctcacctctgaacatgatgggcctgttgctaaggactttctgaacaggctcagaatcatcaaacacaacaaaaccaaaattgggtaatttcccaccactgttaatgcgcaactccaccacgtttccataactttgaaagaaatctttaagctctgatttgtccacttcatgaggcaggttgccaatgaagagttggtgactgtcagggtgtctcaccattcttcggggttcaatgtcaccttgctcaccagcctcacggattggtctgggtcccctttggggaggaatatttattcgttgttctcgcactctttgatcccgctgaggtctttgtggtggaatctgagattcaggcttagactctggacggggctgtgaagctggtactttaacaacatgaggtggtatcccagtaactggaacagctccactgggtggaagattcttactggtcacagatgcccaagaaaatgtcctcaagtcttcctgtactgtctgagctatgtctgcaggtgctggagaagaactcttctgagcatcctcaggggcagtttcttctaatactggctcaggcttttcctcttggatttcagatacaggttcttgttctggttctggttcaggatcaggctctggttcagcaacaggctcctctaaatgttcttccatgtcattactgacaactgcctgatcatagaaagttccagaatcatcaggtaccacctcaggtgtttgctgtctttcttcaggttcctctacttcttcttcagactcctcctgaggctcagtgacaaacccaccaaagacctcatcttggtatctgaagatatcattgtgaacatagaatttatttgcaacagacccctcaggagcaaggacaaacgtttgcatgaatctcctcaaagcctggttgttgttagagagaagccccatcacctggactaccacaccatcatttagcgtggcatgagcatcaacatggcgaatcttggtgtggcagttggtgaagttttgtgacatcactttcctgtggatttctttctgtccgtagactgcatctgctggctttccatttgaatccaatcccccatggacataagaagagttctttccataaaatctatgcagcatgtctggggcctggttcagcagtgtgtaatactgtctcacaaattcccgcccgaccagcaggggactaggcttctccatcaccattgctttggtcaattcaacctggggggaaaagagtcaaatatgtccaaacctacgcggctgagctggagaggaactagctctgcaccacagcaccgaggatagtacaaacccctcacgcaactgcgtccgcac

SEQ ID NO: 13946 - RNA, 884 nt, Homo sapiens
  source 1..884: mol_type = other RNA
gctgggattacaggcatgagccaccccgcccgacccaagttactttttaatagtttaaaaaactgcgtgccaatacaatttcggaatcatataaattactgaccacttgtcacaggattttacaaagagcttcaaatttaggaagataggcaaaacactaggattaatataacaattaaggaaaaaacggctaagaagtgaggttacttgaaaaaataagaggagaaatcaatatgaagctatttcaatgtttacatctataggaaatacaggctgagtattcttaatctgaaaatccaaaatgctccacaatgtgaaattttttgaatgctgacatgatgctcaaagaaaatgctcatcggagcatttcaaacttttgattttttttaattagggatgctcaaccagtacaacacaaatattctaaaacctgaaaaaaaaaaagccaaaatctaaaacacatttctggctcaagcattttggataagggatactcaacttatatatacttcggcttttctaatgttttttagtcttcaaatacagtcttgtcctcatgcaacctgaaatatcttagaaatgccaactttcggcatccacagagccctgtcgacgacaacccacaacatatcttggtccattggtagctttaacaatgaatttttcttcagttaactgtttaagcacttcacccacgatctgcccaacactctgtagggccttcagatcattttcagacttttcatactgcttggtaagttcttttaattgttcccttaactccttaagacggccgtcgatctccttgtgttcaagcaacttcttgcggtagtcctgaagcgccttatctctagggtccgccatgatgagaagccgtctctcat

SEQ ID NO: 13947 - RNA, 8405 nt, Homo sapiens
  source 1..8405: mol_type = other RNA
gctgggattacaggcatgagccacccctcctggcctgggtttaactattttattttatgacagggtctcactttgttgtccaggtaccggtgcgttctctgttcactgcaacctccacctcctgagttcaagcgatcctcccacctcagcctcctgagtagctggaactacagatgcataccaccacacccggctaatttttgtatttgttgtagagacaggttttcactgtgttgcctaggctggtctcaaactcctggtgtcaagggatccactgatctcggcctcccaaagtgctgggattacagaaatgagccaccacgtctggccctgggcttacctttcaagtcaactttgattcattgtcttccttgaaacaccacattcagtgattagtcaaataatgaacattattcttgcacaactcttttgaatctatcaattactttctactcatttagtacatattcactggggagatgctctgtgccagacactgtagtaagatcaggtaattcagaggaagtatagacaccccagacctcaaacgaagacaagataaatatggacaagggaagatccacctccacattcaccattttcagtctttctgtcatttccagctaaataacgtcttcaaaaatgtttcaaaataactaagtcactatttcaaactctttcaataatagcacccttctatacactggactactcttaattttctcattataacatgatcttgcttttcttttaatttttgtctttgctttctacctgaatttttattttgcattatgaaattgataggtccattactggatggcatggttcaattctccagtatgtctgttgatttgtgttccactaaatcttccaattactcagagaggagtgttaatgactgcaactataactggatttttctatttttacttggcgtatccaattttgtttatgagttttgaagctctgtgtcctcatatacatttgggacaatattctcctgaaaaattgacaatcataattatttaggaggcctcattattcctgaaaagtttctctgctttcaaatctactttgtctgattttatatatatacaccacagctgtctttgattaatgcttgcatgaggtatcttttcccactcttttctttcaatctgctctataacttttattcttatttataagtgtattgcaggtggctttctttagtcagcatatttatttttaacacattctgatgatctctagtttttacttaatgcatttagataatttacatataatgttattatagataagtttttagatagatctactatttaataatttattaaccttttttccctttgttttaattcttctatgttcctctgtctatcttgttttggtttatttcaatctggttgttaagtggtctagggattaccatatacatatataacttttcacagtatactaagaatcaatattttaccattcaagttgaatatagaaacttcatcaagagttagtcccattacatttacccttttatcttatgtatgtagtacatctagatacaatgacaactgcatcagataaagttacaatttttgctttcaaccatcaaacataccttaaggaactcaagagaagaataatagtctgttatgtctacccagacattttctatttctgcttttgttccttcattgatgatgttctaagtttccttctggtatcacttttcttatctcaaacctttgctaattcttttccagcagttttgctaggactgagaatgtatttatttaccttccaatgagaatgcatttatttgcctttatgtctggaagatacttttgctccacataccattctgggttgataatgtatttttcctttggtatttactgaatgttatgacatttttttctggctcctgggttcccgatgagaaatctacaatcattcatttggtattttatctttcatttccctttggctgctttcaaaattgttttgtgttttcttaattttccgcagtttgattatgatatgtcttgcaatgggtttcttttggtttatcctgcttgacatttactgaactttaaaaatctggtttatatcttttgagaaatttgatacattttcagccattaattcttcacagttttatcccacaaagacctctttgtcctcttacaataatgtgaatgtttccagattacaataatgtgaatgttagatttgttattttttatttgtccctgagcctctgttcagggacaataaaatcctcctttctttctataggtcagattctgtaggtattcttgttccgttttcaagttcattgactttttccttagtcttctgcatactgctattgagatcatccaattaagctttttatttcccctaatagttttggttaatactttttttaattcttaagtttaaattggtgtttacatattccaaatatttggtgagactttccaactttccattcacttcatgaatgctatcccgtaattctaggagcattgttataataactgctttaatgtatgtgtcagatgattttgacatatgtgtcctctcaatattgttatgcaaggattctctttgccatgtgaattaagatctccctggtttttcataatgctgaatattttggggcttgtaacctggacttctttggattatgtgatgagacactgtgtcttgttgaaatcttaaggataatattgctctttttgtttttgcaggcacacaattgccttgtatttaagctccaagtaccaaccagacttccatgtgttgttgtttcacagataactctatttgaaagccttgacactgcggatgagagatctctggagtgtgtgcaaccagtggtcagtgaggactggaaagtggaccattgtttagttcagtcctcaggctctttttaggtaagttgtttgggattagacccacttattcacagctggcaggtgcgtccacaagctcatgaacaactttatgggtttgctttctacagtatctgtccaggcacattctagttacttgacacatcctggtttcagtcctctcaccagaaagccagggctgtatttacccaggtggctctgccctgcacttttcacagttgcctcacattcaagccgcatttatcgtgtcagctcccgaggtggacaacaggagtctttctgcagcgtcagtgcccatcacacttcctgctgcagaatacatcctccataaacaccatagcatggatgatgacagaggtgaatgaaaagaaagaaaaacattctggtgatgctgtgcaggaaggatctacagtatttgtcaagacattgggtggagagatttgagggagaggagacaaagacactgggaagtcttgagcctagtgtggtagacacaaaagagattctgaattaatagctgatgaatgaatccactcatttatttgtatttgttatgtgaatgaatgttacatgaatgacctggcatggagaaaacagatggtgagactatgtgctagggtaaagcaagagctcaagttttttttttttttttaatttagaaaaaaatctgcttttcatatctggttttcctatttaaaactatgtgatttgaggaaaatggtttaactcctctgagctttagtgtcatctacaaaatttggataatgatactgagggaagctgaaaagccgtatcaaccaacttatacaaaaaataataaacattcacttccatttctaatgcatggtgctgaaaaagtccttgtatgtggaatattgttcacctttaaggaacctgctctcaagagctgatgagggactttttttagtgcagttctgttgtcactggctgttgggctcatttagttggcaccaacaaatctctgtcttgctgctttttttcctcttgtggcccagtcatctagcttttcccttcttcagagatcttagtcactcttcttttccgtagtctccttaaggaactcaagggaagaataatagtctgttatgtctacccagacatgttctatttctgcttttgttccttcactgatgatgttctaagtttccttctggtatcatttttcttatctcaaatctttgctaattcttttccagcagtcttcctaagaatgagaatgtatttacttaccttccactgagaatgcatttatttgcctttatgtctggaagatacttttgctccacatagcattctgggtcgatatgtctttttcttttgttacttaccgaatgttatgacattttttctggcccctatggttcctgatgcgaaatctacaatcattcatttggtagtttctctttcatttccctttggctgctttcaaaattgttttgtattttcttagttttcagcagtttgattatgatatgccttgctatgggtttctttgggtttatcctgattgacatttactgaactttaaaaatctggtttatatcttttgacaaatttgaaccattttcagctattaattgttcaaagttttatcccacaaagaccactttgtcctcttctttccagattacaataatgtgaatgttggatttgttattttttatttgtgcctgagcctctgttcagagacaataaaatcctcctttctctctatagttcagattatgtaggtattcgtgttctgttttcaagttcattgactttttccttagtcttctgcattcgattatggagatcctccaattaagctttttatttcccctaagagttttggttaatacatttttttaattcttaagtttaaattggtgtttatgtattcgaaatatttggtgagactttccaactttccattcacttcacgaatgttatccccgattctaggagcattgttataatatctgctttaatgtatgtgtcagatgattttgacatctgtgtcctctcaatattgttattcgaggattctctttgccatgtgaattaagatctccctgttttttcataatgctgaatattgtggggcttgtaacctggacttctttggattatgtgatgagacactgtgtcttgttgaaatcttaaggataatattgctatttttgtttttgcaggcacacaattgccttgtatttaagctccaagtaccaaccagactttcatgtgttgtcgtttcaaagataactctatttgaaagccttgacactgctgttcagagatctccaaagtgtgtgcaacccagtggtcagtgaggactggaaagtgggccattgcacagttcagctctcaggctctttttaggtaagttgttcgggattagagccacttattcacagctggcaggtgcgtccacaagctcatgaacaactttatggttttgctttctacagtatctgtccaggcacattctagttacttgacacatcttggtttcagtcctctcaccagaaagctggggctgtatttaaccaggtggctctgtcctccacttttcacaattgtctcacatttaggaccaagctgcaggcagaaacagggagaaaagagcagttttatatgtcctttggtttcacagctcctcgaagaaacagaaaattaattacacagtagatctacactatactgaatgccagcaggaagctgtcaccagtcctgtattgttgctgctcctatgtcttgaaccaaagacaccgagagcagtgtcttgctctcagacactgactcgggtttgggtacctaaataataaagcttggagaatgtgggcattgatcccactacctcttgcatgctaagcaagcgctctaccacttgagctaattccccatatcagggaagctttgtttatccttagtgggtggcctggaacacaggtgatttcagggccttcagcgggaaagcagggctctactaagagcagatcttctcattgatggcgcagggcaaggtgcagtggctactcattctctgcaaagaaggaggaaaaaagggaagaaggagaaagtcacaaagggaaaactcacgctgccaaaatgtgaagtttagggtattccaggacagaaaaagacacgtcccagcaaagaagacctatctagacctgcccagctaaagtgtcactgatttttaaaaaataattaaataattaaaaatgattaaatgattgtgtgtgtattgcatgtgtgtgtgtgtgtgtttataaaagtgggatggcattatcacttgttccttgtagctgagactctctgggggttgtgagatggtccagatttctggaaggcacaaaagggattctgaattaatatctgatgaatgaatccactcatttatttgtatttgttatgtgaatgaatgttacaggaatcacctggtgtggagaaaacagatggcaagactatgtgctagggtaaagcaagagctcacgtgtttttgtttttggttttttaatttagaaaaaaaatctgcttttcatatctggttttcctatttaaagctatgtgatttaaggaaaatggtttaactcctctgagctttagtgtcatctacaaaatttggataatgatactgagggaagctgaaaagccatatcaaccaacttatacaaaaaataataaacattcacttccatttctaatgcatggtgctgaaaaagtccttgtatgtggaatattgttcacctttaaggaacctgctctcaagagctgatgcgggactttttttagggcagttctgttgtctctggctgttttgttcatttaattggcacctacaagtctctttgaacattaaaataaaataaagattgtggaggaatagaatacaaacacatagtaaggtgagatttgcataacagagtatagtaaacgatttgtgcctgattctttttgcattctctttgaatcatttttagcctttattctaagtccccaattattgtcatccttttcccaacaagattgtttctctccgccacggacattctggtcagggtctctgcttaaccatcttgacctcctgaacactctgtttgtcctgataacctgatttatgctcaaatgatgctcttccataggacggcttcctgctttgcccaaagagcattcaatttttcaagctgtttagggctccttcctcacccagggtctatttgaaaccttagagggaaggctattctttccaggaagagaaccctgctgggttgtaacctcaatctgtaaatccactggggtaactggggttagctcagttactccagagcttgctctctgagaactggatggtgctgctacttcccataaaggctgaataaaaagaggcatctgcaggcaggagaaagcgctatggtcattgctggaagattccttctgaccattagctatctctctgacctggtgtgagaagggtgacaaaaatcggagacttgaaaacaggccaaaaaaaaaaaaatggattcaaaagaattttaaaagaatcatgcacaagttcttaattagattcttttatccaaatccattttgtctggaaaataataccttactacgtatctgtattctattcctccataatctattttattttattttaatgttcacaagaagctggatgctagctaccaaatgagcaaatcagccacgataacagaactgcactaaaatctctcatcagatattgatacagtcaagaccctcatgagtgcctatgatacaaattcagtgtgagaggccagctttccgcaaggagaaggcaaccaaagcggtagctaatactgagcagttcctattgcccagatccatttctaggtgctgagatccagccagagaatcccacagtcctcatttttcatatgaagaaacatgtgagtgattcaccaccccaatcctcatgtatcatcagttttcaaacaaagccaagtagcctcctgtgcaaaaagctctcctaacccccagttgccttgataggtaaaagtattcttatgacagtgctagaaaaacacgggcacaagtgttccggcaaggtgactagaaggcaaggctaaagttgtcaaggtgacaaagtccctgatggtcctcttgaaagctgaacgtgccacctcatatgtatatgtgtatgtgtggatgcatatgtgtatgttgtgtgtacacacctacacatatatctacaaatgcatgtgtgtatgcatgcatgtgtgtacacgtgcatgcgcacatgtatctgtatacatgtattatgtacacagtatgcatgtgtacatgtatgtgtgtctgtgcatgtgtagatgtatacatgcatgtacacatgcatctacatatgcatgtgtatgcctaaatgtgtgtacaagtgcgtgcatatgtgcactatacatatgtgtacattacgtgtgtgtatgtttctacacgtgtatctgc

SEQ ID NO: 13948 - RNA, 8858 nt, Homo sapiens
  source 1..8858: mol_type = other RNA
gctgggattacaggcatgagccacccctcctggcctgggtttaactattttattttatgacagggtctcactttgttgtccaggtaccggtgcgttctctgttcactgcaacctccacctcctgagttcaagcgatcctcccacctcagcctcctgagtagctggaactacagatgcataccaccacacccggctaatttttgtatttgttgtagagacaggttttcactgtgttgcctaggctggtctcaaactcctggtgtcaagggatccactgatctcggcctcccaaagtgctgggattacagaaatgagccaccacgtctggccctgggcttacctttcaagtcaactttgattcattgtcttccttgaaacaccacattcagtgattagtcaaataatgaacattattcttgcacaactcttttgaatctatcaattactttctactcatttagtacatattcactggggagatgctctgtgccagacactgtagtaagatcaggtaattcagaggaagtatagacaccccagacctcaaacgaagacaagataaatatggacaagggaagatccacctccacattcaccattttcagtctttctgtcatttccagctaaataacgtcttcaaaaatgtttcaaaataactaagtcactatttcaaactctttcaataatagcacccttctatacactggactactcttaattttctcattataacatgatcttgcttttcttttaatttttgtctttgctttctacctgaatttttattttgcattatgaaattgataggtccattactggatggcatggttcaattctccagtatgtctgttgatttgtgttccactaaatcttccaattactcagagaggagtgttaatgactgcaactataactggatttttctatttttacttggcgtatccaattttgtttatgagttttgaagctctgtgtcctcatatacatttgggacaatattctcctgaaaaattgacaatcataattatttaggaggcctcattattcctgaaaagtttctctgctttcaaatctactttgtctgattttatatatatacaccacagctgtctttgattaatgcttgcatgaggtatcttttcccactcttttctttcaatctgctctataacttttattcttatttataagtgtattgcaggtggctttctttagtcagcatatttatttttaacacattctgatgatctctagtttttacttaatgcatttagataatttacatataatgttattatagataagtttttagatagatctactatttaataatttattaaccttttttccctttgttttaattcttctatgttcctctgtctatcttgttttggtttatttcaatctggttgttaagtggtctagggattaccatatacatatataacttttcacagtatactaagaatcaatattttaccattcaagttgaatatagaaacttcatcaagagttagtcccattacatttacccttttatcttatgtatgtagtacatctagatacaatgacaactgcatcagataaagttacaatttttgctttcaaccatcaaacataccttaaggaactcaagagaagaataatagtctgttatgtctacccagacattttctatttctgcttttgttccttcattgatgatgttctaagtttccttctggtatcacttttcttatctcaaacctttgctaattcttttccagcagttttgctaggactgagaatgtatttatttaccttccaatgagaatgcatttatttgcctttatgtctggaagatacttttgctccacataccattctgggttgataatgtatttttcctttggtatttactgaatgttatgacatttttttctggctcctgggttcccgatgagaaatctacaatcattcatttggtattttatctttcatttccctttggctgctttcaaaattgttttgtgttttcttaattttccgcagtttgattatgatatgtcttgcaatgggtttcttttggtttatcctgcttgacatttactgaactttaaaaatctggtttatatcttttgagaaatttgatacattttcagccattaattcttcacagttttatcccacaaagacctctttgtcctcttacaataatgtgaatgtttccagattacaataatgtgaatgttagatttgttattttttatttgtccctgagcctctgttcagggacaataaaatcctcctttctttctataggtcagattctgtaggtattcttgttccgttttcaagttcattgactttttccttagtcttctgcatactgctattgagatcatccaattaagctttttatttcccctaatagttttggttaatactttttttaattcttaagtttaaattggtgtttacatattccaaatatttggtgagactttccaactttccattcacttcatgaatgctatcccgtaattctaggagcattgttataataactgctttaatgtatgtgtcagatgattttgacatatgtgtcctctcaatattgttatgcaaggattctctttgccatgtgaattaagatctccctggtttttcataatgctgaatattttggggcttgtaacctggacttctttggattatgtgatgagacactgtgtcttgttgaaatcttaaggataatattgctctttttgtttttgcaggcacacaattgccttgtatttaagctccaagtaccaaccagacttccatgtgttgttgtttcacagataactctatttgaaagccttgacactgcggatgagagatctctggagtgtgtgcaaccagtggtcagtgaggactggaaagtggaccattgtttagttcagtcctcaggctctttttaggtaagttgtttgggattagacccacttattcacagctggcaggtgcgtccacaagctcatgaacaactttatgggtttgctttctacagtatctgtccaggcacattctagttacttgacacatcctggtttcagtcctctcaccagaaagccagggctgtatttacccaggtggctctgccctgcacttttcacagttgcctcacattcaagctacaggcagaaacagggagaaaagagcaattgtttatgtcccttggtttcacagctcctcaaagaagcagaaaattaattacacggtagatctacactatactgaatgccaggagggagccgtcaccagccctgtattgttgctgctcctacatcttgaaccaaagcagcatcctgttctctgacttgggtttggagacctgagtgtttggagacccagggtctaaataataaagtttggagaatgtgggcatcgatcccactacctcttgcatgctaagcaagcgctctaccacttgagctaattcccccacatcaggggagctttattgatccttagtgggtggcctggaacacaggggatttcagggccttcagcgggaaagcagggctctactaagagcagatcttctcactgatggcccagggcaaggtgcagtggctactcattctccgcatttatcgtgtcagctcccgaggtggacaacaggagtctttctgcagcgtcagtgcccatcacacttcctgctgcagaatacatcctccataaacaccatagcatggatgatgacagaggtgaatgaaaagaaagaaaaacattctggtgatgctgtgcaggaaggatctacagtatttgtcaagacattgggtggagagatttgagggagaggagacaaagacactgggaagtcttgagcctagtgtggtagacacaaaagagattctgaattaatagctgatgaatgaatccactcatttatttgtatttgttatgtgaatgaatgttacatgaatgacctggcatggagaaaacagatggtgagactatgtgctagggtaaagcaagagctcaagttttttttttttttttaatttagaaaaaaatctgcttttcatatctggttttcctatttaaaactatgtgatttgaggaaaatggtttaactcctctgagctttagtgtcatctacaaaatttggataatgatactgagggaagctgaaaagccgtatcaaccaacttatacaaaaaataataaacattcacttccatttctaatgcatggtgctgaaaaagtccttgtatgtggaatattgttcacctttaaggaacctgctctcaagagctgatgagggactttttttagtgcagttctgttgtcactggctgttgggctcatttagttggcaccaacaaatctctgtcttgctgctttttttcctcttgtggcccagtcatctagcttttcccttcttcagagatcttagtcactcttcttttccgtagtctccttaaggaactcaagggaagaataatagtctgttatgtctacccagacatgttctatttctgcttttgttccttcactgatgatgttctaagtttccttctggtatcatttttcttatctcaaatctttgctaattcttttccagcagtcttcctaagaatgagaatgtatttacttaccttccactgagaatgcatttatttgcctttatgtctggaagatacttttgctccacatagcattctgggtcgatatgtctttttcttttgttacttaccgaatgttatgacattttttctggcccctatggttcctgatgcgaaatctacaatcattcatttggtagtttctctttcatttccctttggctgctttcaaaattgttttgtattttcttagttttcagcagtttgattatgatatgccttgctatgggtttctttgggtttatcctgattgacatttactgaactttaaaaatctggtttatatcttttgacaaatttgaaccattttcagctattaattgttcaaagttttatcccacaaagaccactttgtcctcttctttccagattacaataatgtgaatgttggatttgttattttttatttgtgcctgagcctctgttcagagacaataaaatcctcctttctctctatagttcagattatgtaggtattcgtgttctgttttcaagttcattgactttttccttagtcttctgcattcgattatggagatcctccaattaagctttttatttcccctaagagttttggttaatacatttttttaattcttaagtttaaattggtgtttatgtattcgaaatatttggtgagactttccaactttccattcacttcacgaatgttatccccgattctaggagcattgttataatatctgctttaatgtatgtgtcagatgattttgacatctgtgtcctctcaatattgttattcgaggattctctttgccatgtgaattaagatctccctgttttttcataatgctgaatattgtggggcttgtaacctggacttctttggattatgtgatgagacactgtgtcttgttgaaatcttaaggataatattgctatttttgtttttgcaggcacacaattgccttgtatttaagctccaagtaccaaccagactttcatgtgttgtcgtttcaaagataactctatttgaaagccttgacactgctgttcagagatctccaaagtgtgtgcaacccagtggtcagtgaggactggaaagtgggccattgcacagttcagctctcaggctctttttaggtaagttgttcgggattagagccacttattcacagctggcaggtgcgtccacaagctcatgaacaactttatggttttgctttctacagtatctgtccaggcacattctagttacttgacacatcttggtttcagtcctctcaccagaaagctggggctgtatttaaccaggtggctctgtcctccacttttcacaattgtctcacatttaggaccaagctgcaggcagaaacagggagaaaagagcagttttatatgtcctttggtttcacagctcctcgaagaaacagaaaattaattacacagtagatctacactatactgaatgccagcaggaagctgtcaccagtcctgtattgttgctgctcctatgtcttgaaccaaagacaccgagagcagtgtcttgctctcagacactgactcgggtttgggtacctaaataataaagcttggagaatgtgggcattgatcccactacctcttgcatgctaagcaagcgctctaccacttgagctaattccccatatcagggaagctttgtttatccttagtgggtggcctggaacacaggtgatttcagggccttcagcgggaaagcagggctctactaagagcagatcttctcattgatggcgcagggcaaggtgcagtggctactcattctctgcaaagaaggaggaaaaaagggaagaaggagaaagtcacaaagggaaaactcacgctgccaaaatgtgaagtttagggtattccaggacagaaaaagacacgtcccagcaaagaagacctatctagacctgcccagctaaagtgtcactgatttttaaaaaataattaaataattaaaaatgattaaatgattgtgtgtgtattgcatgtgtgtgtgtgtgtgtttataaaagtgggatggcattatcacttgttccttgtagctgagactctctgggggttgtgagatggtccagatttctggaaggcacaaaagggattctgaattaatatctgatgaatgaatccactcatttatttgtatttgttatgtgaatgaatgttacaggaatcacctggtgtggagaaaacagatggcaagactatgtgctagggtaaagcaagagctcacgtgtttttgtttttggttttttaatttagaaaaaaaatctgcttttcatatctggttttcctatttaaagctatgtgatttaaggaaaatggtttaactcctctgagctttagtgtcatctacaaaatttggataatgatactgagggaagctgaaaagccatatcaaccaacttatacaaaaaataataaacattcacttccatttctaatgcatggtgctgaaaaagtccttgtatgtggaatattgttcacctttaaggaacctgctctcaagagctgatgcgggactttttttagggcagttctgttgtctctggctgttttgttcatttaattggcacctacaagtctctttgaacattaaaataaaataaagattgtggaggaatagaatacaaacacatagtaaggtgagatttgcataacagagtatagtaaacgatttgtgcctgattctttttgcattctctttgaatcatttttagcctttattctaagtccccaattattgtcatccttttcccaacaagattgtttctctccgccacggacattctggtcagggtctctgcttaaccatcttgacctcctgaacactctgtttgtcctgataacctgatttatgctcaaatgatgctcttccataggacggcttcctgctttgcccaaagagcattcaatttttcaagctgtttagggctccttcctcacccagggtctatttgaaaccttagagggaaggctattctttccaggaagagaaccctgctgggttgtaacctcaatctgtaaatccactggggtaactggggttagctcagttactccagagcttgctctctgagaactggatggtgctgctacttcccataaaggctgaataaaaagaggcatctgcaggcaggagaaagcgctatggtcattgctggaagattccttctgaccattagctatctctctgacctggtgtgagaagggtgacaaaaatcggagacttgaaaacaggccaaaaaaaaaaaaatggattcaaaagaattttaaaagaatcatgcacaagttcttaattagattcttttatccaaatccattttgtctggaaaataataccttactacgtatctgtattctattcctccataatctattttattttattttaatgttcacaagaagctggatgctagctaccaaatgagcaaatcagccacgataacagaactgcactaaaatctctcatcagatattgatacagtcaagaccctcatgagtgcctatgatacaaattcagtgtgagaggccagctttccgcaaggagaaggcaaccaaagcggtagctaatactgagcagttcctattgcccagatccatttctaggtgctgagatccagccagagaatcccacagtcctcatttttcatatgaagaaacatgtgagtgattcaccaccccaatcctcatgtatcatcagttttcaaacaaagccaagtagcctcctgtgcaaaaagctctcctaacccccagttgccttgataggtaaaagtattcttatgacagtgctagaaaaacacgggcacaagtgttccggcaaggtgactagaaggcaaggctaaagttgtcaaggtgacaaagtccctgatggtcctcttgaaagctgaacgtgccacctcatatgtatatgtgtatgtgtggatgcatatgtgtatgttgtgtgtacacacctacacatatatctacaaatgcatgtgtgtatgcatgcatgtgtgtacacgtgcatgcgcacatgtatctgtatacatgtattatgtacacagtatgcatgtgtacatgtatgtgtgtctgtgcatgtgtagatgtatacatgcatgtacacatgcatctacatatgcatgtgtatgcctaaatgtgtgtacaagtgcgtgcatatgtgcactatacatatgtgtacattacgtgtgtgtatgtttctacacgtgtatctgc

SEQ ID NO: 13949 - RNA, 9527 nt, Homo sapiens
  source 1..9527: mol_type = other RNA
gctgggattacaggcatgagccacccctcctggcctgggtttaactattttattttatgacagggtctcactttgttgtccaggtaccggtgcgttctctgttcactgcaacctccacctcctgagttcaagcgatcctcccacctcagcctcctgagtagctggaactacagatgcataccaccacacccggctaatttttgtatttgttgtagagacaggttttcactgtgttgcctaggctggtctcaaactcctggtgtcaagggatccactgatctcggcctcccaaagtgctgggattacagaaatgagccaccacgtctggccctgggcttacctttcaagtcaactttgattcattgtcttccttgaaacaccacattcagtgattagtcaaataatgaacattattcttgcacaactcttttgaatctatcaattactttctactcatttagtacatattcactggggagatgctctgtgccagacactgtagtaagatcaggtaattcagaggaagtatagacaccccagacctcaaacgaagacaagataaatatggacaagggaagatccacctccacattcaccattttcagtctttctgtcatttccagctaaataacgtcttcaaaaatgtttcaaaataactaagtcactatttcaaactctttcaataatagcacccttctatacactggactactcttaattttctcattataacatgatcttgcttttcttttaatttttgtctttgctttctacctgaatttttattttgcattatgaaattgataggtccattactggatggcatggttcaattctccagtatgtctgttgatttgtgttccactaaatcttccaattactcagagaggagtgttaatgactgcaactataactggatttttctatttttacttggcgtatccaattttgtttatgagttttgaagctctgtgtcctcatatacatttgggacaatattctcctgaaaaattgacaatcataattatttaggaggcctcattattcctgaaaagtttctctgctttcaaatctactttgtctgattttatatatatacaccacagctgtctttgattaatgcttgcatgaggtatcttttcccactcttttctttcaatctgctctataacttttattcttatttataagtgtattgcaggtggctttctttagtcagcatatttatttttaacacattctgatgatctctagtttttacttaatgcatttagataatttacatataatgttattatagataagtttttagatagatctactatttaataatttattaaccttttttccctttgttttaattcttctatgttcctctgtctatcttgttttggtttatttcaatctggttgttaagtggtctagggattaccatatacatatataacttttcacagtatactaagaatcaatattttaccattcaagttgaatatagaaacttcatcaagagttagtcccattacatttacccttttatcttatgtatgtagtacatctagatacaatgacaactgcatcagataaagttacaatttttgctttcaaccatcaaacataccttaaggaactcaagagaagaataatagtctgttatgtctacccagacattttctatttctgcttttgttccttcattgatgatgttctaagtttccttctggtatcacttttcttatctcaaacctttgctaattcttttccagcagttttgctaggactgagaatgtatttatttaccttccaatgagaatgcatttatttgcctttatgtctggaagatacttttgctccacataccattctgggttgataatgtatttttcctttggtatttactgaatgttatgacatttttttctggctcctgggttcccgatgagaaatctacaatcattcatttggtattttatctttcatttccctttggctgctttcaaaattgttttgtgttttcttaattttccgcagtttgattatgatatgtcttgcaatgggtttcttttggtttatcctgcttgacatttactgaactttaaaaatctggtttatatcttttgagaaatttgatacattttcagccattaattcttcacagttttatcccacaaagacctctttgtcctcttacaataatgtgaatgtttccagattacaataatgtgaatgttagatttgttattttttatttgtccctgagcctctgttcagggacaataaaatcctcctttctttctataggtcagattctgtaggtattcttgttccgttttcaagttcattgactttttccttagtcttctgcatactgctattgagatcatccaattaagctttttatttcccctaatagttttggttaatactttttttaattcttaagtttaaattggtgtttacatattccaaatatttggtgagactttccaactttccattcacttcatgaatgctatcccgtaattctaggagcattgttataataactgctttaatgtatgtgtcagatgattttgacatatgtgtcctctcaatattgttatgcaaggattctctttgccatgtgaattaagatctccctggtttttcataatgctgaatattttggggcttgtaacctggacttctttggattatgtgatgagacactgtgtcttgttgaaatcttaaggataatattgctctttttgtttttgcaggcacacaattgccttgtatttaagctccaagtaccaaccagacttccatgtgttgttgtttcacagataactctatttgaaagccttgacactgcggatgagagatctctggagtgtgtgcaaccagtggtcagtgaggactggaaagtggaccattgtttagttcagtcctcaggctctttttaggtaagttgtttgggattagacccacttattcacagctggcaggtgcgtccacaagctcatgaacaactttatgggtttgctttctacagtatctgtccaggcacattctagttacttgacacatcctggtttcagtcctctcaccagaaagccagggctgtatttacccaggtggctctgccctgcacttttcacagttgcctcacattcaagctacaggcagaaacagggagaaaagagcaattgtttatgtcccttggtttcacagctcctcaaagaagcagaaaattaattacacggtagatctacactatactgaatgccaggagggagccgtcaccagccctgtattgttgctgctcctacatcttgaaccaaagcagcatcctgttctctgacttgggtttggagacctgagtgtttggagacccagggtctaaataataaagtttggagaatgtgggcatcgatcccactacctcttgcatgctaagcaagcgctctaccacttgagctaattcccccacatcaggggagctttattgatccttagtgggtggcctggaacacaggggatttcagggccttcagcgggaaagcagggctctactaagagcagatcttctcactgatggcccagggcaaggtgcagtggctactcattctctgcaaagaaggaagaggaaagggaacaaggagaaagtcaaaaagggaaaactcacactgccaaaatgtcaagtttagggtattccgggacagaaaaaggcacattccaggaaaggaggccctgcctagacctgcccatctaaagtgtcactgatttttaaaaaatgattaaataattaaaaatgattaaatgattttgtgtgtgtgtgttgtgtgtgtgtgtttataaaagtgagatagtattatcacttgttccttgtagctgagactctctggggattttgagatggtacagatttctggaaggcaaaaagctcctgttgttttcataactaggccctttcaggaatgaagccagcgtgctgaccactaccttaggaaacccctggggagtgcttctttcacttgcatctgagatataggttgcctccttgctaaggtgtgtcatgtacaagttacatgtccaactatatctcagaacaacaacaacaaaattacagagcagagccataaagaataagagacaagatcatatcagagtgtaagaatatgtaaaatattagagtgtaagaatcaaaattcagctatgcagagaaggagtggacatatggtggagaaaaccgggctgttcgtaggaattcctgtgtgaagaaataaacctgttcaatttaagtgctgtgtgtgtgtgtgtgtgtgtgtgtgtgtgtgaaatacacacggagggaagcagtgattgaaaagcctggccacttggagatatgttggtagagttttatgaaaactcccaagagtaattgaaaaaatcccaggcagaatgcttaaataattaaagcaacatgttagagaaaggtgtttagttttgaatgtcagagcttgaacatgagaaaatagaaattgaagagaaagagaaagaagtcataaagatattaaaggattgagatttacccgcatttatcgtgtcagctcccgaggtggacaacaggagtctttctgcagcgtcagtgcccatcacacttcctgctgcagaatacatcctccataaacaccatagcatggatgatgacagaggtgaatgaaaagaaagaaaaacattctggtgatgctgtgcaggaaggatctacagtatttgtcaagacattgggtggagagatttgagggagaggagacaaagacactgggaagtcttgagcctagtgtggtagacacaaaagagattctgaattaatagctgatgaatgaatccactcatttatttgtatttgttatgtgaatgaatgttacatgaatgacctggcatggagaaaacagatggtgagactatgtgctagggtaaagcaagagctcaagttttttttttttttttaatttagaaaaaaatctgcttttcatatctggttttcctatttaaaactatgtgatttgaggaaaatggtttaactcctctgagctttagtgtcatctacaaaatttggataatgatactgagggaagctgaaaagccgtatcaaccaacttatacaaaaaataataaacattcacttccatttctaatgcatggtgctgaaaaagtccttgtatgtggaatattgttcacctttaaggaacctgctctcaagagctgatgagggactttttttagtgcagttctgttgtcactggctgttgggctcatttagttggcaccaacaaatctctgtcttgctgctttttttcctcttgtggcccagtcatctagcttttcccttcttcagagatcttagtcactcttcttttccgtagtctccgaatgttatgacattttttctggcccctatggttcctgatgcgaaatctacaatcattcatttggtagtttctctttcatttccctttggctgctttcaaaattgttttgtattttcttagttttcagcagtttgattatgatatgccttgctatgggtttctttgggtttatcctgattgacatttactgaactttaaaaatctggtttatatcttttgacaaatttgaaccattttcagctattaattgttcaaagttttatcccacaaagaccactttgtcctcttctttccagattacaataatgtgaatgttggatttgttattttttatttgtgcctgagcctctgttcagagacaataaaatcctcctttctctctatagttcagattatgtaggtattcgtgttctgttttcaagttcattgactttttccttagtcttctgcattcgattatggagatcctccaattaagctttttatttcccctaagagttttggttaatacatttttttaattcttaagtttaaattggtgtttatgtattcgaaatatttggtgagactttccaactttccattcacttcacgaatgttatccccgattctaggagcattgttataatatctgctttaatgtatgtgtcagatgattttgacatctgtgtcctctcaatattgttattcgaggattctctttgccatgtgaattaagatctccctgttttttcataatgctgaatattgtggggcttgtaacctggacttctttggattatgtgatgagacactgtgtcttgttgaaatcttaaggataatattgctatttttgtttttgcaggcacacaattgccttgtatttaagctccaagtaccaaccagactttcatgtgttgtcgtttcaaagataactctatttgaaagccttgacactgctgttcagagatctccaaagtgtgtgcaacccagtggtcagtgaggactggaaagtgggccattgcacagttcagctctcaggctctttttaggtaagttgttcgggattagagccacttattcacagctggcaggtgcgtccacaagctcatgaacaactttatggttttgctttctacagtatctgtccaggcacattctagttacttgacacatcttggtttcagtcctctcaccagaaagctggggctgtatttaaccaggtggctctgtcctccacttttcacaattgtctcacatttaggaccaagctgcaggcagaaacagggagaaaagagcagttttatatgtcctttggtttcacagctcctcgaagaaacagaaaattaattacacagtagatctacactatactgaatgccagcaggaagctgtcaccagtcctgtattgttgctgctcctatgtcttgaaccaaagacaccgagagcagtgtcttgctctcagacactgactcgggtttgggtacctaaataataaagcttggagaatgtgggcattgatcccactacctcttgcatgctaagcaagcgctctaccacttgagctaattccccatatcagggaagctttgtttatccttagtgggtggcctggaacacaggtgatttcagggccttcagcgggaaagcagggctctactaagagcagatcttctcattgatggcgcagggcaaggtgcagtggctactcattctctgcaaagaaggaggaaaaaagggaagaaggagaaagtcacaaagggaaaactcacgctgccaaaatgtgaagtttagggtattccaggacagaaaaagacacgtcccagcaaagaagacctatctagacctgcccagctaaagtgtcactgatttttaaaaaataattaaataattaaaaatgattaaatgattgtgtgtgtattgcatgtgtgtgtgtgtgtgtttataaaagtgggatggcattatcacttgttccttgtagctgagactctctgggggttgtgagatggtccagatttctggaaggcacaaaagggattctgaattaatatctgatgaatgaatccactcatttatttgtatttgttatgtgaatgaatgttacaggaatcacctggtgtggagaaaacagatggcaagactatgtgctagggtaaagcaagagctcacgtgtttttgtttttggttttttaatttagaaaaaaaatctgcttttcatatctggttttcctatttaaagctatgtgatttaaggaaaatggtttaactcctctgagctttagtgtcatctacaaaatttggataatgatactgagggaagctgaaaagccatatcaaccaacttatacaaaaaataataaacattcacttccatttctaatgcatggtgctgaaaaagtccttgtatgtggaatattgttcacctttaaggaacctgctctcaagagctgatgcgggactttttttagggcagttctgttgtctctggctgttttgttcatttaattggcacctacaagtctctttgaacattaaaataaaataaagattgtggaggaatagaatacaaacacatagtaaggtgagatttgcataacagagtatagtaaacgatttgtgcctgattctttttgcattctctttgaatcatttttagcctttattctaagtccccaattattgtcatccttttcccaacaagattgtttctctccgccacggacattctggtcagggtctctgcttaaccatcttgacctcctgaacactctgtttgtcctgataacctgatttatgctcaaatgatgctcttccataggacggcttcctgctttgcccaaagagcattcaatttttcaagctgtttagggctccttcctcacccagggtctatttgaaaccttagagggaaggctattctttccaggaagagaaccctgctgggttgtaacctcaatctgtaaatccactggggtaactggggttagctcagttactccagagcttgctctctgagaactggatggtgctgctacttcccataaaggctgaataaaaagaggcatctgcaggcaggagaaagcgctatggtcattgctggaagattccttctgaccattagctatctctctgacctggtgtgagaagggtgacaaaaatcggagacttgaaaacaggccaaaaaaaaaaaaatggattcaaaagaattttaaaagaatcatgcacaagttcttaattagattcttttatccaaatccattttgtctggaaaataataccttactacgtatctgtattctattcctccataatctattttattttattttaatgttcacaagaagctggatgctagctaccaaatgagcaaatcagccacgataacagaactgcactaaaatctctcatcagatattgatacagtcaagaccctcatgagtgcctatgatacaaattcagtgtgagaggccagctttccgcaaggagaaggcaaccaaagcggtagctaatactgagcagttcctattgcccagatccatttctaggtgctgagatccagccagagaatcccacagtcctcatttttcatatgaagaaacatgtgagtgattcaccaccccaatcctcatgtatcatcagttttcaaacaaagccaagtagcctcctgtgcaaaaagctctcctaacccccagttgccttgataggtaaaagtattcttatgacagtgctagaaaaacacgggcacaagtgttccggcaaggtgactagaaggcaaggctaaagttgtcaaggtgacaaagtccctgatggtcctcttgaaagctgaacgtgccacctcatatgtatatgtgtatgtgtggatgcatatgtgtatgttgtgtgtacacacctacacatatatctacaaatgcatgtgtgtatgcatgcatgtgtgtacacgtgcatgcgcacatgtatctgtatacatgtattatgtacacagtatgcatgtgtacatgtatgtgtgtctgtgcatgtgtagatgtatacatgcatgtacacatgcatctacatatgcatgtgtatgcctaaatgtgtgtacaagtgcgtgcatatgtgcactatacatatgtgtacattacgtgtgtgtatgtttctacacgtgtatctgca

SEQ ID NO: 13950 - RNA, 9681 nt, Homo sapiens
  source 1..9681: mol_type = other RNA
gctgggattacaggcatgagccacccctcctggcctgggtttaactattttattttatgacagggtctcactttgttgtccaggtaccggtgcgttctctgttcactgcaacctccacctcctgagttcaagcgatcctcccacctcagcctcctgagtagctggaactacagatgcataccaccacacccggctaatttttgtatttgttgtagagacaggttttcactgtgttgcctaggctggtctcaaactcctggtgtcaagggatccactgatctcggcctcccaaagtgctgggattacagaaatgagccaccacgtctggccctgggcttacctttcaagtcaactttgattcattgtcttccttgaaacaccacattcagtgattagtcaaataatgaacattattcttgcacaactcttttgaatctatcaattactttctactcatttagtacatattcactggggagatgctctgtgccagacactgtagtaagatcaggtaattcagaggaagtatagacaccccagacctcaaacgaagacaagataaatatggacaagggaagatccacctccacattcaccattttcagtctttctgtcatttccagctaaataacgtcttcaaaaatgtttcaaaataactaagtcactatttcaaactctttcaataatagcacccttctatacactggactactcttaattttctcattataacatgatcttgcttttcttttaatttttgtctttgctttctacctgaatttttattttgcattatgaaattgataggtccattactggatggcatggttcaattctccagtatgtctgttgatttgtgttccactaaatcttccaattactcagagaggagtgttaatgactgcaactataactggatttttctatttttacttggcgtatccaattttgtttatgagttttgaagctctgtgtcctcatatacatttgggacaatattctcctgaaaaattgacaatcataattatttaggaggcctcattattcctgaaaagtttctctgctttcaaatctactttgtctgattttatatatatacaccacagctgtctttgattaatgcttgcatgaggtatcttttcccactcttttctttcaatctgctctataacttttattcttatttataagtgtattgcaggtggctttctttagtcagcatatttatttttaacacattctgatgatctctagtttttacttaatgcatttagataatttacatataatgttattatagataagtttttagatagatctactatttaataatttattaaccttttttccctttgttttaattcttctatgttcctctgtctatcttgttttggtttatttcaatctggttgttaagtggtctagggattaccatatacatatataacttttcacagtatactaagaatcaatattttaccattcaagttgaatatagaaacttcatcaagagttagtcccattacatttacccttttatcttatgtatgtagtacatctagatacaatgacaactgcatcagataaagttacaatttttgctttcaaccatcaaacataccttaaggaactcaagagaagaataatagtctgttatgtctacccagacattttctatttctgcttttgttccttcattgatgatgttctaagtttccttctggtatcacttttcttatctcaaacctttgctaattcttttccagcagttttgctaggactgagaatgtatttatttaccttccaatgagaatgcatttatttgcctttatgtctggaagatacttttgctccacataccattctgggttgataatgtatttttcctttggtatttactgaatgttatgacatttttttctggctcctgggttcccgatgagaaatctacaatcattcatttggtattttatctttcatttccctttggctgctttcaaaattgttttgtgttttcttaattttccgcagtttgattatgatatgtcttgcaatgggtttcttttggtttatcctgcttgacatttactgaactttaaaaatctggtttatatcttttgagaaatttgatacattttcagccattaattcttcacagttttatcccacaaagacctctttgtcctcttacaataatgtgaatgtttccagattacaataatgtgaatgttagatttgttattttttatttgtccctgagcctctgttcagggacaataaaatcctcctttctttctataggtcagattctgtaggtattcttgttccgttttcaagttcattgactttttccttagtcttctgcatactgctattgagatcatccaattaagctttttatttcccctaatagttttggttaatactttttttaattcttaagtttaaattggtgtttacatattccaaatatttggtgagactttccaactttccattcacttcatgaatgctatcccgtaattctaggagcattgttataataactgctttaatgtatgtgtcagatgattttgacatatgtgtcctctcaatattgttatgcaaggattctctttgccatgtgaattaagatctccctggtttttcataatgctgaatattttggggcttgtaacctggacttctttggattatgtgatgagacactgtgtcttgttgaaatcttaaggataatattgctctttttgtttttgcaggcacacaattgccttgtatttaagctccaagtaccaaccagacttccatgtgttgttgtttcacagataactctatttgaaagccttgacactgcggatgagagatctctggagtgtgtgcaaccagtggtcagtgaggactggaaagtggaccattgtttagttcagtcctcaggctctttttaggtaagttgtttgggattagacccacttattcacagctggcaggtgcgtccacaagctcatgaacaactttatgggtttgctttctacagtatctgtccaggcacattctagttacttgacacatcctggtttcagtcctctcaccagaaagccagggctgtatttacccaggtggctctgccctgcacttttcacagttgcctcacattcaagctacaggcagaaacagggagaaaagagcaattgtttatgtcccttggtttcacagctcctcaaagaagcagaaaattaattacacggtagatctacactatactgaatgccaggagggagccgtcaccagccctgtattgttgctgctcctacatcttgaaccaaagcagcatcctgttctctgacttgggtttggagacctgagtgtttggagacccagggtctaaataataaagtttggagaatgtgggcatcgatcccactacctcttgcatgctaagcaagcgctctaccacttgagctaattcccccacatcaggggagctttattgatccttagtgggtggcctggaacacaggggatttcagggccttcagcgggaaagcagggctctactaagagcagatcttctcactgatggcccagggcaaggtgcagtggctactcattctctgcaaagaaggaagaggaaagggaacaaggagaaagtcaaaaagggaaaactcacactgccaaaatgtcaagtttagggtattccgggacagaaaaaggcacattccaggaaaggaggccctgcctagacctgcccatctaaagtgtcactgatttttaaaaaatgattaaataattaaaaatgattaaatgattttgtgtgtgtgtgttgtgtgtgtgtgtttataaaagtgagatagtattatcacttgttccttgtagctgagactctctggggattttgagatggtacagatttctggaaggcaaaaagctcctgttgttttcataactaggccctttcaggaatgaagccagcgtgctgaccactaccttaggaaacccctggggagtgcttctttcacttgcatctgagatataggttgcctccttgctaaggtgtgtcatgtacaagttacatgtccaactatatctcagaacaacaacaacaaaattacagagcagagccataaagaataagagacaagatcatatcagagtgtaagaatatgtaaaatattagagtgtaagaatcaaaattcagctatgcagagaaggagtggacatatggtggagaaaaccgggctgttcgtaggaattcctgtgtgaagaaataaacctgttcaatttaagtgctgtgtgtgtgtgtgtgtgtgtgtgtgtgtgtgaaatacacacggagggaagcagtgattgaaaagcctggccacttggagatatgttggtagagttttatgaaaactcccaagagtaattgaaaaaatcccaggcagaatgcttaaataattaaagcaacatgttagagaaaggtgtttagttttgaatgtcagagcttgaacatgagaaaatagaaattgaagagaaagagaaagaagtcataaagatattaaaggattgagatttacccgcatttatcgtgtcagctcccgaggtggacaacaggagtctttctgcagcgtcagtgcccatcacacttcctgctgcagaatacatcctccataaacaccatagcatggatgatgacagaggtgaatgaaaagaaagaaaaacattctggtgatgctgtgcaggaaggatctacagtatttgtcaagacattgggtggagagatttgagggagaggagacaaagacactgggaagtcttgagcctagtgtggtagacacaaaagagattctgaattaatagctgatgaatgaatccactcatttatttgtatttgttatgtgaatgaatgttacatgaatgacctggcatggagaaaacagatggtgagactatgtgctagggtaaagcaagagctcaagttttttttttttttttaatttagaaaaaaatctgcttttcatatctggttttcctatttaaaactatgtgatttgaggaaaatggtttaactcctctgagctttagtgtcatctacaaaatttggataatgatactgagggaagctgaaaagccgtatcaaccaacttatacaaaaaataataaacattcacttccatttctaatgcatggtgctgaaaaagtccttgtatgtggaatattgttcacctttaaggaacctgctctcaagagctgatgagggactttttttagtgcagttctgttgtcactggctgttgggctcatttagttggcaccaacaaatctctgtcttgctgctttttttcctcttgtggcccagtcatctagcttttcccttcttcagagatcttagtcactcttcttttccgtagtctccttaaggaactcaagggaagaataatagtctgttatgtctacccagacatgttctatttctgcttttgttccttcactgatgatgttctaagtttccttctggtatcatttttcttatctcaaatctttgctaattcttttccagcagtcttccgaatgttatgacattttttctggcccctatggttcctgatgcgaaatctacaatcattcatttggtagtttctctttcatttccctttggctgctttcaaaattgttttgtattttcttagttttcagcagtttgattatgatatgccttgctatgggtttctttgggtttatcctgattgacatttactgaactttaaaaatctggtttatatcttttgacaaatttgaaccattttcagctattaattgttcaaagttttatcccacaaagaccactttgtcctcttctttccagattacaataatgtgaatgttggatttgttattttttatttgtgcctgagcctctgttcagagacaataaaatcctcctttctctctatagttcagattatgtaggtattcgtgttctgttttcaagttcattgactttttccttagtcttctgcattcgattatggagatcctccaattaagctttttatttcccctaagagttttggttaatacatttttttaattcttaagtttaaattggtgtttatgtattcgaaatatttggtgagactttccaactttccattcacttcacgaatgttatccccgattctaggagcattgttataatatctgctttaatgtatgtgtcagatgattttgacatctgtgtcctctcaatattgttattcgaggattctctttgccatgtgaattaagatctccctgttttttcataatgctgaatattgtggggcttgtaacctggacttctttggattatgtgatgagacactgtgtcttgttgaaatcttaaggataatattgctatttttgtttttgcaggcacacaattgccttgtatttaagctccaagtaccaaccagactttcatgtgttgtcgtttcaaagataactctatttgaaagccttgacactgctgttcagagatctccaaagtgtgtgcaacccagtggtcagtgaggactggaaagtgggccattgcacagttcagctctcaggctctttttaggtaagttgttcgggattagagccacttattcacagctggcaggtgcgtccacaagctcatgaacaactttatggttttgctttctacagtatctgtccaggcacattctagttacttgacacatcttggtttcagtcctctcaccagaaagctggggctgtatttaaccaggtggctctgtcctccacttttcacaattgtctcacatttaggaccaagctgcaggcagaaacagggagaaaagagcagttttatatgtcctttggtttcacagctcctcgaagaaacagaaaattaattacacagtagatctacactatactgaatgccagcaggaagctgtcaccagtcctgtattgttgctgctcctatgtcttgaaccaaagacaccgagagcagtgtcttgctctcagacactgactcgggtttgggtacctaaataataaagcttggagaatgtgggcattgatcccactacctcttgcatgctaagcaagcgctctaccacttgagctaattccccatatcagggaagctttgtttatccttagtgggtggcctggaacacaggtgatttcagggccttcagcgggaaagcagggctctactaagagcagatcttctcattgatggcgcagggcaaggtgcagtggctactcattctctgcaaagaaggaggaaaaaagggaagaaggagaaagtcacaaagggaaaactcacgctgccaaaatgtgaagtttagggtattccaggacagaaaaagacacgtcccagcaaagaagacctatctagacctgcccagctaaagtgtcactgatttttaaaaaataattaaataattaaaaatgattaaatgattgtgtgtgtattgcatgtgtgtgtgtgtgtgtttataaaagtgggatggcattatcacttgttccttgtagctgagactctctgggggttgtgagatggtccagatttctggaaggcacaaaagggattctgaattaatatctgatgaatgaatccactcatttatttgtatttgttatgtgaatgaatgttacaggaatcacctggtgtggagaaaacagatggcaagactatgtgctagggtaaagcaagagctcacgtgtttttgtttttggttttttaatttagaaaaaaaatctgcttttcatatctggttttcctatttaaagctatgtgatttaaggaaaatggtttaactcctctgagctttagtgtcatctacaaaatttggataatgatactgagggaagctgaaaagccatatcaaccaacttatacaaaaaataataaacattcacttccatttctaatgcatggtgctgaaaaagtccttgtatgtggaatattgttcacctttaaggaacctgctctcaagagctgatgcgggactttttttagggcagttctgttgtctctggctgttttgttcatttaattggcacctacaagtctctttgaacattaaaataaaataaagattgtggaggaatagaatacaaacacatagtaaggtgagatttgcataacagagtatagtaaacgatttgtgcctgattctttttgcattctctttgaatcatttttagcctttattctaagtccccaattattgtcatccttttcccaacaagattgtttctctccgccacggacattctggtcagggtctctgcttaaccatcttgacctcctgaacactctgtttgtcctgataacctgatttatgctcaaatgatgctcttccataggacggcttcctgctttgcccaaagagcattcaatttttcaagctgtttagggctccttcctcacccagggtctatttgaaaccttagagggaaggctattctttccaggaagagaaccctgctgggttgtaacctcaatctgtaaatccactggggtaactggggttagctcagttactccagagcttgctctctgagaactggatggtgctgctacttcccataaaggctgaataaaaagaggcatctgcaggcaggagaaagcgctatggtcattgctggaagattccttctgaccattagctatctctctgacctggtgtgagaagggtgacaaaaatcggagacttgaaaacaggccaaaaaaaaaaaaatggattcaaaagaattttaaaagaatcatgcacaagttcttaattagattcttttatccaaatccattttgtctggaaaataataccttactacgtatctgtattctattcctccataatctattttattttattttaatgttcacaagaagctggatgctagctaccaaatgagcaaatcagccacgataacagaactgcactaaaatctctcatcagatattgatacagtcaagaccctcatgagtgcctatgatacaaattcagtgtgagaggccagctttccgcaaggagaaggcaaccaaagcggtagctaatactgagcagttcctattgcccagatccatttctaggtgctgagatccagccagagaatcccacagtcctcatttttcatatgaagaaacatgtgagtgattcaccaccccaatcctcatgtatcatcagttttcaaacaaagccaagtagcctcctgtgcaaaaagctctcctaacccccagttgccttgataggtaaaagtattcttatgacagtgctagaaaaacacgggcacaagtgttccggcaaggtgactagaaggcaaggctaaagttgtcaaggtgacaaagtccctgatggtcctcttgaaagctgaacgtgccacctcatatgtatatgtgtatgtgtggatgcatatgtgtatgttgtgtgtacacacctacacatatatctacaaatgcatgtgtgtatgcatgcatgtgtgtacacgtgcatgcgcacatgtatctgtatacatgtattatgtacacagtatgcatgtgtacatgtatgtgtgtctgtgcatgtgtagatgtatacatgcatgtacacatgcatctacatatgcatgtgtatgcctaaatgtgtgtacaagtgcgtgcatatgtgcactatacatatgtgtacattacgtgtgtgtatgtttctacacgtgtatctgcac

SEQ ID NO: 13951 - RNA, 9802 nt, Homo sapiens
  source 1..9802: mol_type = other RNA
gctgggattacaggcatgagccacccctcctggcctgggtttaactattttattttatgacagggtctcactttgttgtccaggtaccggtgcgttctctgttcactgcaacctccacctcctgagttcaagcgatcctcccacctcagcctcctgagtagctggaactacagatgcataccaccacacccggctaatttttgtatttgttgtagagacaggttttcactgtgttgcctaggctggtctcaaactcctggtgtcaagggatccactgatctcggcctcccaaagtgctgggattacagaaatgagccaccacgtctggccctgggcttacctttcaagtcaactttgattcattgtcttccttgaaacaccacattcagtgattagtcaaataatgaacattattcttgcacaactcttttgaatctatcaattactttctactcatttagtacatattcactggggagatgctctgtgccagacactgtagtaagatcaggtaattcagaggaagtatagacaccccagacctcaaacgaagacaagataaatatggacaagggaagatccacctccacattcaccattttcagtctttctgtcatttccagctaaataacgtcttcaaaaatgtttcaaaataactaagtcactatttcaaactctttcaataatagcacccttctatacactggactactcttaattttctcattataacatgatcttgcttttcttttaatttttgtctttgctttctacctgaatttttattttgcattatgaaattgataggtccattactggatggcatggttcaattctccagtatgtctgttgatttgtgttccactaaatcttccaattactcagagaggagtgttaatgactgcaactataactggatttttctatttttacttggcgtatccaattttgtttatgagttttgaagctctgtgtcctcatatacatttgggacaatattctcctgaaaaattgacaatcataattatttaggaggcctcattattcctgaaaagtttctctgctttcaaatctactttgtctgattttatatatatacaccacagctgtctttgattaatgcttgcatgaggtatcttttcccactcttttctttcaatctgctctataacttttattcttatttataagtgtattgcaggtggctttctttagtcagcatatttatttttaacacattctgatgatctctagtttttacttaatgcatttagataatttacatataatgttattatagataagtttttagatagatctactatttaataatttattaaccttttttccctttgttttaattcttctatgttcctctgtctatcttgttttggtttatttcaatctggttgttaagtggtctagggattaccatatacatatataacttttcacagtatactaagaatcaatattttaccattcaagttgaatatagaaacttcatcaagagttagtcccattacatttacccttttatcttatgtatgtagtacatctagatacaatgacaactgcatcagataaagttacaatttttgctttcaaccatcaaacataccttaaggaactcaagagaagaataatagtctgttatgtctacccagacattttctatttctgcttttgttccttcattgatgatgttctaagtttccttctggtatcacttttcttatctcaaacctttgctaattcttttccagcagttttgctaggactgagaatgtatttatttaccttccaatgagaatgcatttatttgcctttatgtctggaagatacttttgctccacataccattctgggttgataatgtatttttcctttggtatttactgaatgttatgacatttttttctggctcctgggttcccgatgagaaatctacaatcattcatttggtattttatctttcatttccctttggctgctttcaaaattgttttgtgttttcttaattttccgcagtttgattatgatatgtcttgcaatgggtttcttttggtttatcctgcttgacatttactgaactttaaaaatctggtttatatcttttgagaaatttgatacattttcagccattaattcttcacagttttatcccacaaagacctctttgtcctcttacaataatgtgaatgtttccagattacaataatgtgaatgttagatttgttattttttatttgtccctgagcctctgttcagggacaataaaatcctcctttctttctataggtcagattctgtaggtattcttgttccgttttcaagttcattgactttttccttagtcttctgcatactgctattgagatcatccaattaagctttttatttcccctaatagttttggttaatactttttttaattcttaagtttaaattggtgtttacatattccaaatatttggtgagactttccaactttccattcacttcatgaatgctatcccgtaattctaggagcattgttataataactgctttaatgtatgtgtcagatgattttgacatatgtgtcctctcaatattgttatgcaaggattctctttgccatgtgaattaagatctccctggtttttcataatgctgaatattttggggcttgtaacctggacttctttggattatgtgatgagacactgtgtcttgttgaaatcttaaggataatattgctctttttgtttttgcaggcacacaattgccttgtatttaagctccaagtaccaaccagacttccatgtgttgttgtttcacagataactctatttgaaagccttgacactgcggatgagagatctctggagtgtgtgcaaccagtggtcagtgaggactggaaagtggaccattgtttagttcagtcctcaggctctttttaggtaagttgtttgggattagacccacttattcacagctggcaggtgcgtccacaagctcatgaacaactttatgggtttgctttctacagtatctgtccaggcacattctagttacttgacacatcctggtttcagtcctctcaccagaaagccagggctgtatttacccaggtggctctgccctgcacttttcacagttgcctcacattcaagctacaggcagaaacagggagaaaagagcaattgtttatgtcccttggtttcacagctcctcaaagaagcagaaaattaattacacggtagatctacactatactgaatgccaggagggagccgtcaccagccctgtattgttgctgctcctacatcttgaaccaaagcagcatcctgttctctgacttgggtttggagacctgagtgtttggagacccagggtctaaataataaagtttggagaatgtgggcatcgatcccactacctcttgcatgctaagcaagcgctctaccacttgagctaattcccccacatcaggggagctttattgatccttagtgggtggcctggaacacaggggatttcagggccttcagcgggaaagcagggctctactaagagcagatcttctcactgatggcccagggcaaggtgcagtggctactcattctctgcaaagaaggaagaggaaagggaacaaggagaaagtcaaaaagggaaaactcacactgccaaaatgtcaagtttagggtattccgggacagaaaaaggcacattccaggaaaggaggccctgcctagacctgcccatctaaagtgtcactgatttttaaaaaatgattaaataattaaaaatgattaaatgattttgtgtgtgtgtgttgtgtgtgtgtgtttataaaagtgagatagtattatcacttgttccttgtagctgagactctctggggattttgagatggtacagatttctggaaggcaaaaagctcctgttgttttcataactaggccctttcaggaatgaagccagcgtgctgaccactaccttaggaaacccctggggagtgcttctttcacttgcatctgagatataggttgcctccttgctaaggtgtgtcatgtacaagttacatgtccaactatatctcagaacaacaacaacaaaattacagagcagagccataaagaataagagacaagatcatatcagagtgtaagaatatgtaaaatattagagtgtaagaatcaaaattcagctatgcagagaaggagtggacatatggtggagaaaaccgggctgttcgtaggaattcctgtgtgaagaaataaacctgttcaatttaagtgctgtgtgtgtgtgtgtgtgtgtgtgtgtgtgtgaaatacacacggagggaagcagtgattgaaaagcctggccacttggagatatgttggtagagttttatgaaaactcccaagagtaattgaaaaaatcccaggcagaatgcttaaataattaaagcaacatgttagagaaaggtgtttagttttgaatgtcagagcttgaacatgagaaaatagaaattgaagagaaagagaaagaagtcataaagatattaaaggattgagatttacccgcatttatcgtgtcagctcccgaggtggacaacaggagtctttctgcagcgtcagtgcccatcacacttcctgctgcagaatacatcctccataaacaccatagcatggatgatgacagaggtgaatgaaaagaaagaaaaacattctggtgatgctgtgcaggaaggatctacagtatttgtcaagacattgggtggagagatttgagggagaggagacaaagacactgggaagtcttgagcctagtgtggtagacacaaaagagattctgaattaatagctgatgaatgaatccactcatttatttgtatttgttatgtgaatgaatgttacatgaatgacctggcatggagaaaacagatggtgagactatgtgctagggtaaagcaagagctcaagttttttttttttttttaatttagaaaaaaatctgcttttcatatctggttttcctatttaaaactatgtgatttgaggaaaatggtttaactcctctgagctttagtgtcatctacaaaatttggataatgatactgagggaagctgaaaagccgtatcaaccaacttatacaaaaaataataaacattcacttccatttctaatgcatggtgctgaaaaagtccttgtatgtggaatattgttcacctttaaggaacctgctctcaagagctgatgagggactttttttagtgcagttctgttgtcactggctgttgggctcatttagttggcaccaacaaatctctgtcttgctgctttttttcctcttgtggcccagtcatctagcttttcccttcttcagagatcttagtcactcttcttttccgtagtctccttaaggaactcaagggaagaataatagtctgttatgtctacccagacatgttctatttctgcttttgttccttcactgatgatgttctaagtttccttctggtatcatttttcttatctcaaatctttgctaattcttttccagcagtcttcctaagaatgagaatgtatttacttaccttccactgagaatgcatttatttgcctttatgtctggaagatacttttgctccacatagcattctgggtcgatatgtctttttcttttgttacttaccgaatgttatgacattttttctggcccctatggttcctgatgcgaaatctacaatcattcatttggtagtttctctttcatttccctttggctgctttcaaaattgttttgtattttcttagttttcagcagtttgattatgatatgccttgctatgggtttctttgggtttatcctgattgacatttactgaactttaaaaatctggtttatatcttttgacaaatttgaaccattttcagctattaattgttcaaagttttatcccacaaagaccactttgtcctcttctttccagattacaataatgtgaatgttggatttgttattttttatttgtgcctgagcctctgttcagagacaataaaatcctcctttctctctatagttcagattatgtaggtattcgtgttctgttttcaagttcattgactttttccttagtcttctgcattcgattatggagatcctccaattaagctttttatttcccctaagagttttggttaatacatttttttaattcttaagtttaaattggtgtttatgtattcgaaatatttggtgagactttccaactttccattcacttcacgaatgttatccccgattctaggagcattgttataatatctgctttaatgtatgtgtcagatgattttgacatctgtgtcctctcaatattgttattcgaggattctctttgccatgtgaattaagatctccctgttttttcataatgctgaatattgtggggcttgtaacctggacttctttggattatgtgatgagacactgtgtcttgttgaaatcttaaggataatattgctatttttgtttttgcaggcacacaattgccttgtatttaagctccaagtaccaaccagactttcatgtgttgtcgtttcaaagataactctatttgaaagccttgacactgctgttcagagatctccaaagtgtgtgcaacccagtggtcagtgaggactggaaagtgggccattgcacagttcagctctcaggctctttttaggtaagttgttcgggattagagccacttattcacagctggcaggtgcgtccacaagctcatgaacaactttatggttttgctttctacagtatctgtccaggcacattctagttacttgacacatcttggtttcagtcctctcaccagaaagctggggctgtatttaaccaggtggctctgtcctccacttttcacaattgtctcacatttaggaccaagctgcaggcagaaacagggagaaaagagcagttttatatgtcctttggtttcacagctcctcgaagaaacagaaaattaattacacagtagatctacactatactgaatgccagcaggaagctgtcaccagtcctgtattgttgctgctcctatgtcttgaaccaaagacaccgagagcagtgtcttgctctcagacactgactcgggtttgggtacctaaataataaagcttggagaatgtgggcattgatcccactacctcttgcatgctaagcaagcgctctaccacttgagctaattccccatatcagggaagctttgtttatccttagtgggtggcctggaacacaggtgatttcagggccttcagcgggaaagcagggctctactaagagcagatcttctcattgatggcgcagggcaaggtgcagtggctactcattctctgcaaagaaggaggaaaaaagggaagaaggagaaagtcacaaagggaaaactcacgctgccaaaatgtgaagtttagggtattccaggacagaaaaagacacgtcccagcaaagaagacctatctagacctgcccagctaaagtgtcactgatttttaaaaaataattaaataattaaaaatgattaaatgattgtgtgtgtattgcatgtgtgtgtgtgtgtgtttataaaagtgggatggcattatcacttgttccttgtagctgagactctctgggggttgtgagatggtccagatttctggaaggcacaaaagggattctgaattaatatctgatgaatgaatccactcatttatttgtatttgttatgtgaatgaatgttacaggaatcacctggtgtggagaaaacagatggcaagactatgtgctagggtaaagcaagagctcacgtgtttttgtttttggttttttaatttagaaaaaaaatctgcttttcatatctggttttcctatttaaagctatgtgatttaaggaaaatggtttaactcctctgagctttagtgtcatctacaaaatttggataatgatactgagggaagctgaaaagccatatcaaccaacttatacaaaaaataataaacattcacttccatttctaatgcatggtgctgaaaaagtccttgtatgtggaatattgttcacctttaaggaacctgctctcaagagctgatgcgggactttttttagggcagttctgttgtctctggctgttttgttcatttaattggcacctacaagtctctttgaacattaaaataaaataaagattgtggaggaatagaatacaaacacatagtaaggtgagatttgcataacagagtatagtaaacgatttgtgcctgattctttttgcattctctttgaatcatttttagcctttattctaagtccccaattattgtcatccttttcccaacaagattgtttctctccgccacggacattctggtcagggtctctgcttaaccatcttgacctcctgaacactctgtttgtcctgataacctgatttatgctcaaatgatgctcttccataggacggcttcctgctttgcccaaagagcattcaatttttcaagctgtttagggctccttcctcacccagggtctatttgaaaccttagagggaaggctattctttccaggaagagaaccctgctgggttgtaacctcaatctgtaaatccactggggtaactggggttagctcagttactccagagcttgctctctgagaactggatggtgctgctacttcccataaaggctgaataaaaagaggcatctgcaggcaggagaaagcgctatggtcattgctggaagattccttctgaccattagctatctctctgacctggtgtgagaagggtgacaaaaatcggagacttgaaaacaggccaaaaaaaaaaaaatggattcaaaagaattttaaaagaatcatgcacaagttcttaattagattcttttatccaaatccattttgtctggaaaataataccttactacgtatctgtattctattcctccataatctattttattttattttaatgttcacaagaagctggatgctagctaccaaatgagcaaatcagccacgataacagaactgcactaaaatctctcatcagatattgatacagtcaagaccctcatgagtgcctatgatacaaattcagtgtgagaggccagctttccgcaaggagaaggcaaccaaagcggtagctaatactgagcagttcctattgcccagatccatttctaggtgctgagatccagccagagaatcccacagtcctcatttttcatatgaagaaacatgtgagtgattcaccaccccaatcctcatgtatcatcagttttcaaacaaagccaagtagcctcctgtgcaaaaagctctcctaacccccagttgccttgataggtaaaagtattcttatgacagtgctagaaaaacacgggcacaagtgttccggcaaggtgactagaaggcaaggctaaagttgtcaaggtgacaaagtccctgatggtcctcttgaaagctgaacgtgccacctcatatgtatatgtgtatgtgtggatgcatatgtgtatgttgtgtgtacacacctacacatatatctacaaatgcatgtgtgtatgcatgcatgtgtgtacacgtgcatgcgcacatgtatctgtatacatgtattatgtacacagtatgcatgtgtacatgtatgtgtgtctgtgcatgtgtagatgtatacatgcatgtacacatgcatctacatatgcatgtgtatgcctaaatgtgtgtacaagtgcgtgcatatgtgcactatacatatgtgtacattacgtgtgtgtatgtttctacacgtgtatctg

SEQ ID NO: 13952 - RNA, 5440 nt, Homo sapiens
  source 1..5440: mol_type = other RNA
gctgggattacaggcatgagccacccctcctggcctgggtttaactattttattttatgacagggtctcactttgttgtccaggtaccggtgcgttctctgttcactgcaacctccacctcctgagttcaagcgatcctcccacctcagcctcctgagtagctggaactacagatgcataccaccacacccggctaatttttgtatttgttgtagagacaggttttcactgtgttgcctaggctggtctcaaactcctggtgtcaagggatccactgatctcggcctcccaaagtgctgggattacagaaatgagccaccacgtctggccctgggcttacctttcaagtcaactttgattcattgtcttccttgaaacaccacattcagtgattagtcaaataatgaacattattcttgcacaactcttttgaatctatcaattactttctactcatttagtacatattcactggggagatgctctgtgccagacactgtagtaagatcaggtaattcagaggaagtatagacaccccagacctcaaacgaagacaagataaatatggacaagggaagatccacctccacattcaccattttcagtctttctgtcatttccagctaaataacgtcttcaaaaatgtttcaaaataactaagtcactatttcaaactctttcaataatagcacccttctatacactggactactcttaattttctcattataacatgatcttgcttttcttttaatttttgtctttgctttctacctgaatttttattttgcattatgaaattgataggtccattactggatggcatggttcaattctccagtatgtctgttgatttgtgttccactaaatcttccaattactcagagaggagtgttaatgactgcaactataactggatttttctatttttacttggcgtatccaattttgtttatgagttttgaagctctgtgtcctcatatacatttgggacaatattctcctgaaaaattgacaatcataattatttaggaggcctcattattcctgaaaagtttctctgctttcaaatctactttgtctgattttatatatatacaccacagctgtctttgattaatgcttgcatgaggtatcttttcccactcttttctttcaatctgctctataacttttattcttatttataagtgtattgcaggtggctttctttagtcagcatatttatttttaacacattctgatgatctctagtttttacttaatgcatttagataatttacatataatgttattatagataagtttttagatagatctactatttaataatttattaaccttttttccctttgttttaattcttctatgttcctctgtctatcttgttttggtttatttcaatctggttgttaagtggtctagggattaccatatacatatataacttttcacagtatactaagaatcaatattttaccattcaagttgaatatagaaacttcatcaagagttagtcccattacatttacccttttatcttatgtatgtagtacatctagatacaatgacaactgcatcagataaagttacaatttttgctttcaaccatcaaacataccttaaggaactcaagagaagaataatagtctgttatgtctacccagacattttctatttctgcttttgttccttcattgatgatgttctaagtttccttctggtatcacttttcttatctcaaacctttgctaattcttttccagcagttttgctaggactgagaatgtatttatttaccttccaatgagaatgcatttatttgcctttatgtctggaagatacttttgctccacataccattctgggttgataatgtatttttcctttggtatttactgaatgttatgacatttttttctggctcctgggttcccgatgagaaatctacaatcattcatttggtattttatctttcatttccctttggctgctttcaaaattgttttgtgttttcttaattttccgcagtttgattatgatatgtcttgcaatgggtttcttttggtttatcctgcttgacatttactgaactttaaaaatctggtttatatcttttgagaaatttgatacattttcagccattaattcttcacagttttatcccacaaagacctctttgtcctcttacaataatgtgaatgtttccagattacaataatgtgaatgttagatttgttattttttatttgtccctgagcctctgttcagggacaataaaatcctcctttctttctataggtcagattctgtaggtattcttgttccgttttcaagttcattgactttttccttagtcttctgcatactgctattgagatcatccaattaagctttttatttcccctaatagttttggttaatactttttttaattcttaagtttaaattggtgtttacatattccaaatatttggtgagactttccaactttccattcacttcatgaatgctatcccgtaattctaggagcattgttataataactgctttaatgtatgtgtcagatgattttgacatatgtgtcctctcaatattgttatgcaaggattctctttgccatgtgaattaagatctccctggtttttcataatgctgaatattttggggcttgtaacctggacttctttggattatgtgatgagacactgtgtcttgttgaaatcttaaggataatattgctctttttgtttttgcaggcacacaattgccttgtatttaagctccaagtaccaaccagacttccatgtgttgttgtttcacagataactctatttgaaagccttgacactgcggatgagagatctctggagtgtgtgcaaccagtggtcagtgaggactggaaagtggaccattgtttagttcagtcctcaggctctttttaggtaagttgtttgggattagacccacttattcacagctggcaggtgcgtccacaagctcatgaacaactttatgggtttgctttctacagtatctgtccaggcacattctagttacttgacacatcctggtttcagtcctctcaccagaaagccagggctgtatttacccaggtggctctgccctgcacttttcacagttgcctcacattcaagctacaggcagaaacagggagaaaagagcaattgtttatgtcccttggtttcacagctcctcaaagaagcagaaaattaattacacggtagatctacactatactgaatgccaggagggagccgtcaccagccctgtattgttgctgctcctacatcttgaaccaaagcagcatcctgttctctgacttgggtttggagacctgagtgtttggagacccagggtctaaataataaagtttggagaatgtgggcatcgatcccactacctcttgcatgctaagcaagcgctctaccacttgagctaattcccccacatcaggggagctttattgatccttagtgggtggcctggaacacaggggatttcagggccttcagcgggaaagcagggctctactaagagcagatcttctcactgatggcccagggcaaggtgcagtggctactcattctctgcaaagaaggaagaggaaagggaacaaggagaaagtcaaaaagggaaaactcacactgccaaaatgtcaagtttagggtattccgggacagaaaaaggcacattccaggaaaggaggccctgcctagacctgcccatctaaagtgtcactgatttttaaaaaatgattaaataattaaaaatgattaaatgattttgtgtgtgtgtgttgtgtgtgtgtgtttataaaagtgagatagtattatcacttgttccttgtagctgagactctctggggattttgagatggtacagatttctggaaggcaaaaagctcctgttgttttcataactaggccctttcaggaatgaagccagcgtgctgaccactaccttaggaaacccctggggagtgcttctttcacttgcatctgagatataggttgcctccttgctaaggtgtgtcatgtacaagttacatgtccaactatatctcagaacaacaacaacaaaattacagagcagagccataaagaataagagacaagatcatatcagagtgtaagaatatgtaaaatattagagtgtaagaatcaaaattcagctatgcagagaaggagtggacatatggtggagaaaaccgggctgttcgtaggaattcctgtgtgaagaaataaacctgttcaatttaagtgctgtgtgtgtgtgtgtgtgtgtgtgtgtgtgtgaaatacacacggagggaagcagtgattgaaaagcctggccacttggagatatgttggtagagttttatgaaaactcccaagagtaattgaaaaaatcccaggcagaatgcttaaataattaaagcaacatgttagagaaaggtgtttagttttgaatgtcagagcttgaacatgagaaaatagaaattgaagagaaagagaaagaagtcataaagatattaaaggattgagatttacccgcatttatcgtgtcagctcccgaggtggacaacaggagtctttctgcagcgtcagtgcccatcacacttcctgctgcagaatacatcctccataaacaccatagcatggatgatgacagaggtgaatgaaaagaaagaaaaacattctggtgatgctgtgcaggaaggatctacagtatttgtcaagacattgggtggagagatttgagggagaggagacaaagacactgggaagtcttgagcctagtgtggtagacacaaaagagattctgaattaatagctgatgaatgaatccactcatttatttgtatttgttatgtgaatgaatgttacatgaatgacctggcatggagaaaacagatggtgagactatgtgctagggtaaagcaagagctcaagttttttttttttttttaatttagaaaaaaatctgcttttcatatctggttttcctatttaaaactatgtgatttgaggaaaatggtttaactcctctgagctttagtgtcatctacaaaatttggataatgatactgagggaagctgaaaagccgtatcaaccaacttatacaaaaaataataaacattcacttccatttctaatgcatggtgctgaaaaagtccttgtatgtggaatattgttcacctttaaggaacctgctctcaagagctgatgagggactttttttagtgcagttctgttgtcactggctgttgggctcatttagttggcaccaacaaatctctgtcttgctgctttttttcctcttgtggcccagtcatctagcttttcccttcttcagagatcttagtcactcttcttttccgtagtctctttgttgtccaggcaccggtgcaatctctgttcactgcaacctccg

SEQ ID NO: 13953 - RNA, 9299 nt, Homo sapiens
  source 1..9299: mol_type = other RNA
gctgggattacaggcatgagccacccctcctggcctgggtttaactattttattttatgacagggtctcactttgttgtccaggtaccggtgcgttctctgttcactgcaacctccacctcctgagttcaagcgatcctcccacctcagcctcctgagtagctggaactacagatgcataccaccacacccggctaatttttgtatttgttgtagagacaggttttcactgtgttgcctaggctggtctcaaactcctggtgtcaagggatccactgatctcggcctcccaaagtgctgggattacagaaatgagccaccacgtctggccctgggcttacctttcaagtcaactttgattcattgtcttccttgaaacaccacattcagtgattagtcaaataatgaacattattcttgcacaactcttttgaatctatcaattactttctactcatttagtacatattcactggggagatgctctgtgccagacactgtagtaagatcaggtaattcagaggaagtatagacaccccagacctcaaacgaagacaagataaatatggacaagggaagatccacctccacattcaccattttcagtctttctgtcatttccagctaaataacgtcttcaaaaatgtttcaaaataactaagtcactatttcaaactctttcaataatagcacccttctatacactggactactcttaattttctcattataacatgatcttgcttttcttttaatttttgtctttgctttctacctgaatttttattttgcattatgaaattgataggtccattactggatggcatggttcaattctccagtatgtctgttgatttgtgttccactaaatcttccaattactcagagaggagtgttaatgactgcaactataactggatttttctatttttacttggcgtatccaattttgtttatgagttttgaagctctgtgtcctcatatacatttgggacaatattctcctgaaaaattgacaatcataattatttaggaggcctcattattcctgaaaagtttctctgctttcaaatctactttgtctgattttatatatatacaccacagctgtctttgattaatgcttgcatgaggtatcttttcccactcttttctttcaatctgctctataacttttattcttatttataagtgtattgcaggtggctttctttagtcagcatatttatttttaacacattctgatgatctctagtttttacttaatgcatttagataatttacatataatgttattatagataagtttttagatagatctactatttaataatttattaaccttttttccctttgttttaattcttctatgttcctctgtctatcttgttttggtttatttcaatctggttgttaagtggtctagggattaccatatacatatataacttttcacagtatactaagaatcaatattttaccattcaagttgaatatagaaacttcatcaagagttagtcccattacatttacccttttatcttatgtatgtagtacatctagatacaatgacaactgcatcagataaagttacaatttttgctttcaaccatcaaacataccttaaggaactcaagagaagaataatagtctgttatgtctacccagacattttctatttctgcttttgttccttcattgatgatgttctaagtttccttctggtatcacttttcttatctcaaacctttgctaattcttttccagcagttttgctaggactgagaatgtatttatttaccttccaatgagaatgcatttatttgcctttatgtctggaagatacttttgctccacataccattctgggttgataatgtatttttcctttggtatttactgaatgttatgacatttttttctggctcctgggttcccgatgagaaatctacaatcattcatttggtattttatctttcatttccctttggctgctttcaaaattgttttgtgttttcttaattttccgcagtttgattatgatatgtcttgcaatgggtttcttttggtttatcctgcttgacatttactgaactttaaaaatctggtttatatcttttgagaaatttgatacattttcagccattaattcttcacagttttatcccacaaagacctctttgtcctcttacaataatgtgaatgtttccagattacaataatgtgaatgttagatttgttattttttatttgtccctgagcctctgttcagggacaataaaatcctcctttctttctataggtcagattctgtaggtattcttgttccgttttcaagttcattgactttttccttagtcttctgcatactgctattgagatcatccaattaagctttttatttcccctaatagttttggttaatactttttttaattcttaagtttaaattggtgtttacatattccaaatatttggtgagactttccaactttccattcacttcatgaatgctatcccgtaattctaggagcattgttataataactgctttaatgtatgtgtcagatgattttgacatatgtgtcctctcaatattgttatgcaaggattctctttgccatgtgaattaagatctccctggtttttcataatgctgaatattttggggcttgtaacctggacttctttggattatgtgatgagacactgtgtcttgttgaaatcttaaggataatattgctctttttgtttttgcaggcacacaattgccttgtatttaagctccaagtaccaaccagacttccatgtgttgttgtttcacagataactctatttgaaagccttgacactgcggatgagagatctctggagtgtgtgcaaccagtggtcagtgaggactggaaagtggaccattgtttagttcagtcctcaggctctttttaggtaagttgtttgggattagacccacttattcacagctggcaggtgcgtccacaagctcatgaacaactttatgggtttgctttctacagtatctgtccaggcacattctagttacttgacacatcctggtttcagtcctctcaccagaaagccagggctgtatttacccaggtggctctgccctgcacttttcacagttgcctcacattcaagctacaggcagaaacagggagaaaagagcaattgtttatgtcccttggtttcacagctcctcaaagaagcagaaaattaattacacggtagatctacactatactgaatgccaggagggagccgtcaccagccctgtattgttgctgctcctacatcttgaaccaaagcagcatcctgttctctgacttgggtttggagacctgagtgtttggagacccagggtctaaataataaagtttggagaatgtgggcatcgatcccactacctcttgcatgctaagcaagcgctctaccacttgagctaattcccccacatcaggggagctttattgatccttagtgggtggcctggaacacaggggatttcagggccttcagcgggaaagcagggctctactaagagcagatcttctcactgatggcccagggcaaggtgcagtggctactcattctctgcaaagaaggaagaggaaagggaacaaggagaaagtcaaaaagggaaaactcacactgccaaaatgtcaagtttagggtattccgggacagaaaaaggcacattccaggaaaggaggccctgcctagacctgcccatctaaagtgtcactgatttttaaaaaatgattaaataattaaaaatgattaaatgattttgtgtgtgtgtgttgtgtgtgtgtgtttataaaagtgagatagtattatcacttgttccttgtagctgagactctctggggattttgagatggtacagatttctggaaggcaaaaagctcctgttgttttcataactaggccctttcaggaatgaagccagcgtgctgaccactaccttaggaaacccctggggagtgcttctttcacttgcatctgagatataggttgcctccttgctaaggtgtgtcatgtacaagttacatgtccaactatatctcagaacaacaacaacaaaattacagagcagagccataaagaataagagacaagatcatatcagagtgtaagaatatgtaaaatattagagtgtaagaatcaaaattcagctatgcagagaaggagtggacatatggtggagaaaaccgggctgttcgtaggaattcctgtgtgaagaaataaacctgttcaatttaagtgctgtgtgtgtgtgtgtgtgtgtgtgtgtgtgtgaaatacacacggagggaagcagtgattgaaaagcctggccacttggagatatgttggtagagttttatgaaaactcccaagagtaattgaaaaaatcccaggcagaatgcttaaataattaaagcaacatgttagagaaaggtgtttagttttgaatgtcagagcttgaacatgagaaaatagaaattgaagagaaagagaaagaagtcataaagatattaaaggattgagatttacccgcatttatcgtgtcagctcccgaggtggacaacaggagtctttctgcagcgtcagtgcccatcacacttcctgctgcagaatacatcctccataaacaccatagcatggatgatgacagaggtgaatgaaaagaaagaaaaacattctggtgatgctgtgcaggaaggatctacagtatttgtcaagacattgggtggagagatttgagggagaggagacaaagacactgggaagtcttgagcctgtcttgctgctttttttcctcttgtggcccagtcatctagcttttcccttcttcagagatcttagtcactcttcttttccgtagtctccttaaggaactcaagggaagaataatagtctgttatgtctacccagacatgttctatttctgcttttgttccttcactgatgatgttctaagtttccttctggtatcatttttcttatctcaaatctttgctaattcttttccagcagtcttcctaagaatgagaatgtatttacttaccttccactgagaatgcatttatttgcctttatgtctggaagatacttttgctccacatagcattctgggtcgatatgtctttttcttttgttacttaccgaatgttatgacattttttctggcccctatggttcctgatgcgaaatctacaatcattcatttggtagtttctctttcatttccctttggctgctttcaaaattgttttgtattttcttagttttcagcagtttgattatgatatgccttgctatgggtttctttgggtttatcctgattgacatttactgaactttaaaaatctggtttatatcttttgacaaatttgaaccattttcagctattaattgttcaaagttttatcccacaaagaccactttgtcctcttctttccagattacaataatgtgaatgttggatttgttattttttatttgtgcctgagcctctgttcagagacaataaaatcctcctttctctctatagttcagattatgtaggtattcgtgttctgttttcaagttcattgactttttccttagtcttctgcattcgattatggagatcctccaattaagctttttatttcccctaagagttttggttaatacatttttttaattcttaagtttaaattggtgtttatgtattcgaaatatttggtgagactttccaactttccattcacttcacgaatgttatccccgattctaggagcattgttataatatctgctttaatgtatgtgtcagatgattttgacatctgtgtcctctcaatattgttattcgaggattctctttgccatgtgaattaagatctccctgttttttcataatgctgaatattgtggggcttgtaacctggacttctttggattatgtgatgagacactgtgtcttgttgaaatcttaaggataatattgctatttttgtttttgcaggcacacaattgccttgtatttaagctccaagtaccaaccagactttcatgtgttgtcgtttcaaagataactctatttgaaagccttgacactgctgttcagagatctccaaagtgtgtgcaacccagtggtcagtgaggactggaaagtgggccattgcacagttcagctctcaggctctttttaggtaagttgttcgggattagagccacttattcacagctggcaggtgcgtccacaagctcatgaacaactttatggttttgctttctacagtatctgtccaggcacattctagttacttgacacatcttggtttcagtcctctcaccagaaagctggggctgtatttaaccaggtggctctgtcctccacttttcacaattgtctcacatttaggaccaagctgcaggcagaaacagggagaaaagagcagttttatatgtcctttggtttcacagctcctcgaagaaacagaaaattaattacacagtagatctacactatactgaatgccagcaggaagctgtcaccagtcctgtattgttgctgctcctatgtcttgaaccaaagacaccgagagcagtgtcttgctctcagacactgactcgggtttgggtacctaaataataaagcttggagaatgtgggcattgatcccactacctcttgcatgctaagcaagcgctctaccacttgagctaattccccatatcagggaagctttgtttatccttagtgggtggcctggaacacaggtgatttcagggccttcagcgggaaagcagggctctactaagagcagatcttctcattgatggcgcagggcaaggtgcagtggctactcattctctgcaaagaaggaggaaaaaagggaagaaggagaaagtcacaaagggaaaactcacgctgccaaaatgtgaagtttagggtattccaggacagaaaaagacacgtcccagcaaagaagacctatctagacctgcccagctaaagtgtcactgatttttaaaaaataattaaataattaaaaatgattaaatgattgtgtgtgtattgcatgtgtgtgtgtgtgtgtttataaaagtgggatggcattatcacttgttccttgtagctgagactctctgggggttgtgagatggtccagatttctggaaggcacaaaagggattctgaattaatatctgatgaatgaatccactcatttatttgtatttgttatgtgaatgaatgttacaggaatcacctggtgtggagaaaacagatggcaagactatgtgctagggtaaagcaagagctcacgtgtttttgtttttggttttttaatttagaaaaaaaatctgcttttcatatctggttttcctatttaaagctatgtgatttaaggaaaatggtttaactcctctgagctttagtgtcatctacaaaatttggataatgatactgagggaagctgaaaagccatatcaaccaacttatacaaaaaataataaacattcacttccatttctaatgcatggtgctgaaaaagtccttgtatgtggaatattgttcacctttaaggaacctgctctcaagagctgatgcgggactttttttagggcagttctgttgtctctggctgttttgttcatttaattggcacctacaagtctctttgaacattaaaataaaataaagattgtggaggaatagaatacaaacacatagtaaggtgagatttgcataacagagtatagtaaacgatttgtgcctgattctttttgcattctctttgaatcatttttagcctttattctaagtccccaattattgtcatccttttcccaacaagattgtttctctccgccacggacattctggtcagggtctctgcttaaccatcttgacctcctgaacactctgtttgtcctgataacctgatttatgctcaaatgatgctcttccataggacggcttcctgctttgcccaaagagcattcaatttttcaagctgtttagggctccttcctcacccagggtctatttgaaaccttagagggaaggctattctttccaggaagagaaccctgctgggttgtaacctcaatctgtaaatccactggggtaactggggttagctcagttactccagagcttgctctctgagaactggatggtgctgctacttcccataaaggctgaataaaaagaggcatctgcaggcaggagaaagcgctatggtcattgctggaagattccttctgaccattagctatctctctgacctggtgtgagaagggtgacaaaaatcggagacttgaaaacaggccaaaaaaaaaaaaatggattcaaaagaattttaaaagaatcatgcacaagttcttaattagattcttttatccaaatccattttgtctggaaaataataccttactacgtatctgtattctattcctccataatctattttattttattttaatgttcacaagaagctggatgctagctaccaaatgagcaaatcagccacgataacagaactgcactaaaatctctcatcagatattgatacagtcaagaccctcatgagtgcctatgatacaaattcagtgtgagaggccagctttccgcaaggagaaggcaaccaaagcggtagctaatactgagcagttcctattgcccagatccatttctaggtgctgagatccagccagagaatcccacagtcctcatttttcatatgaagaaacatgtgagtgattcaccaccccaatcctcatgtatcatcagttttcaaacaaagccaagtagcctcctgtgcaaaaagctctcctaacccccagttgccttgataggtaaaagtattcttatgacagtgctagaaaaacacgggcacaagtgttccggcaaggtgactagaaggcaaggctaaagttgtcaaggtgacaaagtccctgatggtcctcttgaaagctgaacgtgccacctcatatgtatatgtgtatgtgtggatgcatatgtgtatgttgtgtgtacacacctacacatatatctacaaatgcatgtgtgtatgcatgcatgtgtgtacacgtgcatgcgcacatgtatctgtatacatgtattatgtacacagtatgcatgtgtacatgtatgtgtgtctgtgcatgtgtagatgtatacatgcatgtacacatgcatctacatatgcatgtgtatgcctaaatgtgtgtacaagtgcgtgcatatgtgcactatacatatgtgtacattacgtgtgtgtatgtttctacacgtgtatctg

SEQ ID NO: 13954 - RNA, 9143 nt, Homo sapiens
  source 1..9143: mol_type = other RNA
gctgggattacaggcatgagccacccctcctggcctgggtttaactattttattttatgacagggtctcactttgttgtccaggtaccggtgcgttctctgttcactgcaacctccacctcctgagttcaagcgatcctcccacctcagcctcctgagtagctggaactacagatgcataccaccacacccggctaatttttgtatttgttgtagagacaggttttcactgtgttgcctaggctggtctcaaactcctggtgtcaagggatccactgatctcggcctcccaaagtgctgggattacagaaatgagccaccacgtctggccctgggcttacctttcaagtcaactttgattcattgtcttccttgaaacaccacattcagtgattagtcaaataatgaacattattcttgcacaactcttttgaatctatcaattactttctactcatttagtacatattcactggggagatgctctgtgccagacactgtagtaagatcaggtaattcagaggaagtatagacaccccagacctcaaacgaagacaagataaatatggacaagggaagatccacctccacattcaccattttcagtctttctgtcatttccagctaaataacgtcttcaaaaatgtttcaaaataactaagtcactatttcaaactctttcaataatagcacccttctatacactggactactcttaattttctcattataacatgatcttgcttttcttttaatttttgtctttgctttctacctgaatttttattttgcattatgaaattgataggtccattactggatggcatggttcaattctccagtatgtctgttgatttgtgttccactaaatcttccaattactcagagaggagtgttaatgactgcaactataactggatttttctatttttacttggcgtatccaattttgtttatgagttttgaagctctgtgtcctcatatacatttgggacaatattctcctgaaaaattgacaatcataattatttaggaggcctcattattcctgaaaagtttctctgctttcaaatctactttgtctgattttatatatatacaccacagctgtctttgattaatgcttgcatgaggtatcttttcccactcttttctttcaatctgctctataacttttattcttatttataagtgtattgcaggtggctttctttagtcagcatatttatttttaacacattctgatgatctctagtttttacttaatgcatttagataatttacatataatgttattatagataagtttttagatagatctactatttaataatttattaaccttttttccctttgttttaattcttctatgttcctctgtctatcttgttttggtttatttcaatctggttgttaagtggtctagggattaccatatacatatataacttttcacagtatactaagaatcaatattttaccattcaagttgaatatagaaacttcatcaagagttagtcccattacatttacccttttatcttatgtatgtagtacatctagatacaatgacaactgcatcagataaagttacaatttttgctttcaaccatcaaacataccttaaggaactcaagagaagaataatagtctgttatgtctacccagacattttctatttctgcttttgttccttcattgatgatgttctaagtttccttctggtatcacttttcttatctcaaacctttgctaattcttttccagcagttttgctaggactgagaatgtatttatttaccttccaatgagaatgcatttatttgcctttatgtctggaagatacttttgctccacataccattctgggttgataatgtatttttcctttggtatttactgaatgttatgacatttttttctggctcctgggttcccgatgagaaatctacaatcattcatttggtattttatctttcatttccctttggctgctttcaaaattgttttgtgttttcttaattttccgcagtttgattatgatatgtcttgcaatgggtttcttttggtttatcctgcttgacatttactgaactttaaaaatctggtttatatcttttgagaaatttgatacattttcagccattaattcttcacagttttatcccacaaagacctctttgtcctcttacaataatgtgaatgtttccagattacaataatgtgaatgttagatttgttattttttatttgtccctgagcctctgttcagggacaataaaatcctcctttctttctataggtcagattctgtaggtattcttgttccgttttcaagttcattgactttttccttagtcttctgcatactgctattgagatcatccaattaagctttttatttcccctaatagttttggttaatactttttttaattcttaagtttaaattggtgtttacatattccaaatatttggtgagactttccaactttccattcacttcatgaatgctatcccgtaattctaggagcattgttataataactgctttaatgtatgtgtcagatgattttgacatatgtgtcctctcaatattgttatgcaaggattctctttgccatgtgaattaagatctccctggtttttcataatgctgaatattttggggcttgtaacctggacttctttggattatgtgatgagacactgtgtcttgttgaaatcttaaggataatattgctctttttgtttttgcaggcacacaattgccttgtatttaagctccaagtaccaaccagacttccatgtgttgttgtttcacagataactctatttgaaagccttgacactgcggatgagagatctctggagtgtgtgcaaccagtggtcagtgaggactggaaagtggaccattgtttagttcagtcctcaggctctttttaggtaagttgtttgggattagacccacttattcacagctggcaggtgcgtccacaagctcatgaacaactttatgggtttgctttctacagtatctgtccaggcacattctagttacttgacacatcctggtttcagtcctctcaccagaaagccagggctgtatttacccaggtggctctgccctgcacttttcacagttgcctcacattcaagctacaggcagaaacagggagaaaagagcaattgtttatgtcccttggtttcacagctcctcaaagaagcagaaaattaattacacggtagatctacactatactgaatgccaggagggagccgtcaccagccctgtattgttgctgctcctacatcttgaaccaaagcagcatcctgttctctgacttgggtttggagacctgagtgtttggagacccagggtctaaataataaagtttggagaatgtgggcatcgatcccactacctcttgcatgctaagcaagcgctctaccacttgagctaattcccccacatcaggggagctttattgatccttagtgggtggcctggaacacaggggatttcagggccttcagcgggaaagcagggctctactaagagcagatcttctcactgatggcccagggcaaggtgcagtggctactcattctctgcaaagaaggaagaggaaagggaacaaggagaaagtcaaaaagggaaaactcacactgccaaaatgtcaagtttagggtattccgggacagaaaaaggcacattccaggaaaggaggccctgcctagacctgcccatctaaagtgtcactgatttttaaaaaatgattaaataattaaaaatgattaaatgattttgtgtgtgtgtgttgtgtgtgtgtgtttataaaagtgagatagtattatcacttgttccttgtagctgagactctctggggattttgagatggtacagatttctggaaggcaaaaagctcctgttgttttcataactaggccctttcaggaatgaagccagcgtgctgaccactaccttaggaaacccctggggagtgcttctttcacttgcatctgagatataggttgcctccttgctaaggtgtgtcatgtacaagttacatgtccaactatatctcagaacaacaacaacaaaattacagagcagagccataaagaataagagacaagatcatatcagagtgtaagaatatgtaaaatattagagtgtaagaatcaaaattcagctatgcagagaaggagtggacatatggtggagaaaaccgggctgttcgtaggaattcctgtgtgaagaaataaacctgttcaatttaagtgctgtgtgtgtgtgtgtgtgtgtgtgtgtgtgtgaaatacacacggagggaagcagtgattgaaaagcctggccacttggagatatgttggtagagttttatgaaaactcccaagagtaattgaaaaaatcccaggcagaatgcttaaataattaaagcaacatgttagagaaaggtgtttagttttgaatgtcagagcttgaacatgagaaaatagaaattgaagagaaagagaaagaagtcataaagatattaaaggattgagatttacccgcatttatcgtgtcagctcccgaggtggacaacaggagtctttctgcagcgtcagtgcccatcacacttcctgctgcagaatacatcctgtcttgctgctttttttcctcttgtggcccagtcatctagcttttcccttcttcagagatcttagtcactcttcttttccgtagtctccttaaggaactcaagggaagaataatagtctgttatgtctacccagacatgttctatttctgcttttgttccttcactgatgatgttctaagtttccttctggtatcatttttcttatctcaaatctttgctaattcttttccagcagtcttcctaagaatgagaatgtatttacttaccttccactgagaatgcatttatttgcctttatgtctggaagatacttttgctccacatagcattctgggtcgatatgtctttttcttttgttacttaccgaatgttatgacattttttctggcccctatggttcctgatgcgaaatctacaatcattcatttggtagtttctctttcatttccctttggctgctttcaaaattgttttgtattttcttagttttcagcagtttgattatgatatgccttgctatgggtttctttgggtttatcctgattgacatttactgaactttaaaaatctggtttatatcttttgacaaatttgaaccattttcagctattaattgttcaaagttttatcccacaaagaccactttgtcctcttctttccagattacaataatgtgaatgttggatttgttattttttatttgtgcctgagcctctgttcagagacaataaaatcctcctttctctctatagttcagattatgtaggtattcgtgttctgttttcaagttcattgactttttccttagtcttctgcattcgattatggagatcctccaattaagctttttatttcccctaagagttttggttaatacatttttttaattcttaagtttaaattggtgtttatgtattcgaaatatttggtgagactttccaactttccattcacttcacgaatgttatccccgattctaggagcattgttataatatctgctttaatgtatgtgtcagatgattttgacatctgtgtcctctcaatattgttattcgaggattctctttgccatgtgaattaagatctccctgttttttcataatgctgaatattgtggggcttgtaacctggacttctttggattatgtgatgagacactgtgtcttgttgaaatcttaaggataatattgctatttttgtttttgcaggcacacaattgccttgtatttaagctccaagtaccaaccagactttcatgtgttgtcgtttcaaagataactctatttgaaagccttgacactgctgttcagagatctccaaagtgtgtgcaacccagtggtcagtgaggactggaaagtgggccattgcacagttcagctctcaggctctttttaggtaagttgttcgggattagagccacttattcacagctggcaggtgcgtccacaagctcatgaacaactttatggttttgctttctacagtatctgtccaggcacattctagttacttgacacatcttggtttcagtcctctcaccagaaagctggggctgtatttaaccaggtggctctgtcctccacttttcacaattgtctcacatttaggaccaagctgcaggcagaaacagggagaaaagagcagttttatatgtcctttggtttcacagctcctcgaagaaacagaaaattaattacacagtagatctacactatactgaatgccagcaggaagctgtcaccagtcctgtattgttgctgctcctatgtcttgaaccaaagacaccgagagcagtgtcttgctctcagacactgactcgggtttgggtacctaaataataaagcttggagaatgtgggcattgatcccactacctcttgcatgctaagcaagcgctctaccacttgagctaattccccatatcagggaagctttgtttatccttagtgggtggcctggaacacaggtgatttcagggccttcagcgggaaagcagggctctactaagagcagatcttctcattgatggcgcagggcaaggtgcagtggctactcattctctgcaaagaaggaggaaaaaagggaagaaggagaaagtcacaaagggaaaactcacgctgccaaaatgtgaagtttagggtattccaggacagaaaaagacacgtcccagcaaagaagacctatctagacctgcccagctaaagtgtcactgatttttaaaaaataattaaataattaaaaatgattaaatgattgtgtgtgtattgcatgtgtgtgtgtgtgtgtttataaaagtgggatggcattatcacttgttccttgtagctgagactctctgggggttgtgagatggtccagatttctggaaggcacaaaagggattctgaattaatatctgatgaatgaatccactcatttatttgtatttgttatgtgaatgaatgttacaggaatcacctggtgtggagaaaacagatggcaagactatgtgctagggtaaagcaagagctcacgtgtttttgtttttggttttttaatttagaaaaaaaatctgcttttcatatctggttttcctatttaaagctatgtgatttaaggaaaatggtttaactcctctgagctttagtgtcatctacaaaatttggataatgatactgagggaagctgaaaagccatatcaaccaacttatacaaaaaataataaacattcacttccatttctaatgcatggtgctgaaaaagtccttgtatgtggaatattgttcacctttaaggaacctgctctcaagagctgatgcgggactttttttagggcagttctgttgtctctggctgttttgttcatttaattggcacctacaagtctctttgaacattaaaataaaataaagattgtggaggaatagaatacaaacacatagtaaggtgagatttgcataacagagtatagtaaacgatttgtgcctgattctttttgcattctctttgaatcatttttagcctttattctaagtccccaattattgtcatccttttcccaacaagattgtttctctccgccacggacattctggtcagggtctctgcttaaccatcttgacctcctgaacactctgtttgtcctgataacctgatttatgctcaaatgatgctcttccataggacggcttcctgctttgcccaaagagcattcaatttttcaagctgtttagggctccttcctcacccagggtctatttgaaaccttagagggaaggctattctttccaggaagagaaccctgctgggttgtaacctcaatctgtaaatccactggggtaactggggttagctcagttactccagagcttgctctctgagaactggatggtgctgctacttcccataaaggctgaataaaaagaggcatctgcaggcaggagaaagcgctatggtcattgctggaagattccttctgaccattagctatctctctgacctggtgtgagaagggtgacaaaaatcggagacttgaaaacaggccaaaaaaaaaaaaatggattcaaaagaattttaaaagaatcatgcacaagttcttaattagattcttttatccaaatccattttgtctggaaaataataccttactacgtatctgtattctattcctccataatctattttattttattttaatgttcacaagaagctggatgctagctaccaaatgagcaaatcagccacgataacagaactgcactaaaatctctcatcagatattgatacagtcaagaccctcatgagtgcctatgatacaaattcagtgtgagaggccagctttccgcaaggagaaggcaaccaaagcggtagctaatactgagcagttcctattgcccagatccatttctaggtgctgagatccagccagagaatcccacagtcctcatttttcatatgaagaaacatgtgagtgattcaccaccccaatcctcatgtatcatcagttttcaaacaaagccaagtagcctcctgtgcaaaaagctctcctaacccccagttgccttgataggtaaaagtattcttatgacagtgctagaaaaacacgggcacaagtgttccggcaaggtgactagaaggcaaggctaaagttgtcaaggtgacaaagtccctgatggtcctcttgaaagctgaacgtgccacctcatatgtatatgtgtatgtgtggatgcatatgtgtatgttgtgtgtacacacctacacatatatctacaaatgcatgtgtgtatgcatgcatgtgtgtacacgtgcatgcgcacatgtatctgtatacatgtattatgtacacagtatgcatgtgtacatgtatgtgtgtctgtgcatgtgtagatgtatacatgcatgtacacatgcatctacatatgcatgtgtatgcctaaatgtgtgtacaagtgcgtgcatatgtgcactatacatatgtgtacattacgtgtgtgtatgtttctacacgtgtatctg

SEQ ID NO: 13955 - RNA, 8109 nt, Homo sapiens
  source 1..8109: mol_type = other RNA
gctgggattacaggcatgagccacccctcctggcctgggtttaactattttattttatgacagggtctcactttgttgtccaggtaccggtgcgttctctgttcactgcaacctccacctcctgagttcaagcgatcctcccacctcagcctcctgagtagctggaactacagatgcataccaccacacccggctaatttttgtatttgttgtagagacaggttttcactgtgttgcctaggctggtctcaaactcctggtgtcaagggatccactgatctcggcctcccaaagtgctgggattacagaaatgagccaccacgtctggccctgggcttacctttcaagtcaactttgattcattgtcttccttgaaacaccacattcagtgattagtcaaataatgaacattattcttgcacaactcttttgaatctatcaattactttctactcatttagtacatattcactggggagatgctctgtgccagacactgtagtaagatcaggtaattcagaggaagtatagacaccccagacctcaaacgaagacaagataaatatggacaagggaagatccacctccacattcaccattttcagtctttctgtcatttccagctaaataacgtcttcaaaaatgtttcaaaataactaagtcactatttcaaactctttcaataatagcacccttctatacactggactactcttaattttctcattataacatgatcttgcttttcttttaatttttgtctttgctttctacctgaatttttattttgcattatgaaattgataggtccattactggatggcatggttcaattctccagtatgtctgttgatttgtgttccactaaatcttccaattactcagagaggagtgttaatgactgcaactataactggatttttctatttttacttggcgtatccaattttgtttatgagttttgaagctctgtgtcctcatatacatttgggacaatattctcctgaaaaattgacaatcataattatttaggaggcctcattattcctgaaaagtttctctgctttcaaatctactttgtctgattttatatatatacaccacagctgtctttgattaatgcttgcatgaggtatcttttcccactcttttctttcaatctgctctataacttttattcttatttataagtgtattgcaggtggctttctttagtcagcatatttatttttaacacattctgatgatctctagtttttacttaatgcatttagataatttacatataatgttattatagataagtttttagatagatctactatttaataatttattaaccttttttccctttgttttaattcttctatgttcctctgtctatcttgttttggtttatttcaatctggttgttaagtggtctagggattaccatatacatatataacttttcacagtatactaagaatcaatattttaccattcaagttgaatatagaaacttcatcaagagttagtcccattacatttacccttttatcttatgtatgtagtacatctagatacaatgacaactgcatcagataaagttacaatttttgctttcaaccatcaaacataccttaaggaactcaagagaagaataatagtctgttatgtctacccagacattttctatttctgcttttgttccttcattgatgatgttctaagtttccttctggtatcacttttcttatctcaaacctttgctaattcttttccagcagttttgctaggactgagaatgtatttatttaccttccaatgagaatgcatttatttgcctttatgtctggaagatacttttgctccacataccattctgggttgataatgtatttttcctttggtatttactgaatgttatgacatttttttctggctcctgggttcccgatgagaaatctacaatcattcatttggtattttatctttcatttccctttggctgctttcaaaattgttttgtgttttcttaattttccgcagtttgattatgatatgtcttgcaatgggtttcttttggtttatcctgcttgacatttactgaactttaaaaatctggtttatatcttttgagaaatttgatacattttcagccattaattcttcacagttttatcccacaaagacctctttgtcctcttacaataatgtgaatgtttccagattacaataatgtgaatgttagatttgttattttttatttgtccctgagcctctgttcagggacaataaaatcctcctttctttctataggtcagattctgtaggtattcttgttccgttttcaagttcattgactttttccttagtcttctgcatactgctattgagatcatccaattaagctttttatttcccctaatagttttggttaatactttttttaattcttaagtttaaattggtgtttacatattccaaatatttggtgagactttccaactttccattcacttcatgaatgctatcccgtaattctaggagcattgttataataactgctttaatgtatgtgtcagatgattttgacatatgtgtcctctcaatattgttatgcaaggattctctttgccatgtgaattaagatctccctggtttttcataatgctgaatattttggggcttgtaacctggacttctttggattatgtgatgagacactgtgtcttgttgaaatcttaaggataatattgctctttttgtttttgcaggcacacaattgccttgtatttaagctccaagtaccaaccagacttccatgtgttgttgtttcacagataactctatttgaaagccttgacactgcggatgagagatctctggagtgtgtgcaaccagtggtcagtgaggactggaaagtggaccattgtttagttcagtcctcaggctctttttaggtaagttgtttgggattagacccacttattcacagctggcaggtgcgtccacaagctcatgaacaactttatgggtttgctttctacagtatctgtccaggcacattctagttacttgacacatcctggtttcagtcctctcaccagaaagccagggctgtatttacccaggtggctctgccctgcacttttcacagttgcctcacattcaagctacaggcagaaacagggagaaaagagcaattgtttatgtcccttggtttcacagctcctcaaagaagcagaaaattaattacacggtagatctacactatactgaatgccaggagggagccgtcaccagccctgtattgttgctgctcctacatcttgaaccaaagcagcatcctgttctctgacttgggtttggagacctgagtgtttggagacccagggtctaaataataaagtttggagaatgtgggcatcgatcccactacctcttgcatgctaagcaagcgctctaccacttgagctaattcccccacatcaggggagctttattgatccttagtgggtggcctggaacacaggggatttcagggccttcagcgggaaagcagggctctactaagagcagatcttctcactgatggcccagggcaaggtgcagtggctactcattctctgtcttgctgctttttttcctcttgtggcccagtcatctagcttttcccttcttcagagatcttagtcactcttcttttccgtagtctccttaaggaactcaagggaagaataatagtctgttatgtctacccagacatgttctatttctgcttttgttccttcactgatgatgttctaagtttccttctggtatcatttttcttatctcaaatctttgctaattcttttccagcagtcttcctaagaatgagaatgtatttacttaccttccactgagaatgcatttatttgcctttatgtctggaagatacttttgctccacatagcattctgggtcgatatgtctttttcttttgttacttaccgaatgttatgacattttttctggcccctatggttcctgatgcgaaatctacaatcattcatttggtagtttctctttcatttccctttggctgctttcaaaattgttttgtattttcttagttttcagcagtttgattatgatatgccttgctatgggtttctttgggtttatcctgattgacatttactgaactttaaaaatctggtttatatcttttgacaaatttgaaccattttcagctattaattgttcaaagttttatcccacaaagaccactttgtcctcttctttccagattacaataatgtgaatgttggatttgttattttttatttgtgcctgagcctctgttcagagacaataaaatcctcctttctctctatagttcagattatgtaggtattcgtgttctgttttcaagttcattgactttttccttagtcttctgcattcgattatggagatcctccaattaagctttttatttcccctaagagttttggttaatacatttttttaattcttaagtttaaattggtgtttatgtattcgaaatatttggtgagactttccaactttccattcacttcacgaatgttatccccgattctaggagcattgttataatatctgctttaatgtatgtgtcagatgattttgacatctgtgtcctctcaatattgttattcgaggattctctttgccatgtgaattaagatctccctgttttttcataatgctgaatattgtggggcttgtaacctggacttctttggattatgtgatgagacactgtgtcttgttgaaatcttaaggataatattgctatttttgtttttgcaggcacacaattgccttgtatttaagctccaagtaccaaccagactttcatgtgttgtcgtttcaaagataactctatttgaaagccttgacactgctgttcagagatctccaaagtgtgtgcaacccagtggtcagtgaggactggaaagtgggccattgcacagttcagctctcaggctctttttaggtaagttgttcgggattagagccacttattcacagctggcaggtgcgtccacaagctcatgaacaactttatggttttgctttctacagtatctgtccaggcacattctagttacttgacacatcttggtttcagtcctctcaccagaaagctggggctgtatttaaccaggtggctctgtcctccacttttcacaattgtctcacatttaggaccaagctgcaggcagaaacagggagaaaagagcagttttatatgtcctttggtttcacagctcctcgaagaaacagaaaattaattacacagtagatctacactatactgaatgccagcaggaagctgtcaccagtcctgtattgttgctgctcctatgtcttgaaccaaagacaccgagagcagtgtcttgctctcagacactgactcgggtttgggtacctaaataataaagcttggagaatgtgggcattgatcccactacctcttgcatgctaagcaagcgctctaccacttgagctaattccccatatcagggaagctttgtttatccttagtgggtggcctggaacacaggtgatttcagggccttcagcgggaaagcagggctctactaagagcagatcttctcattgatggcgcagggcaaggtgcagtggctactcattctctgcaaagaaggaggaaaaaagggaagaaggagaaagtcacaaagggaaaactcacgctgccaaaatgtgaagtttagggtattccaggacagaaaaagacacgtcccagcaaagaagacctatctagacctgcccagctaaagtgtcactgatttttaaaaaataattaaataattaaaaatgattaaatgattgtgtgtgtattgcatgtgtgtgtgtgtgtgtttataaaagtgggatggcattatcacttgttccttgtagctgagactctctgggggttgtgagatggtccagatttctggaaggcacaaaagggattctgaattaatatctgatgaatgaatccactcatttatttgtatttgttatgtgaatgaatgttacaggaatcacctggtgtggagaaaacagatggcaagactatgtgctagggtaaagcaagagctcacgtgtttttgtttttggttttttaatttagaaaaaaaatctgcttttcatatctggttttcctatttaaagctatgtgatttaaggaaaatggtttaactcctctgagctttagtgtcatctacaaaatttggataatgatactgagggaagctgaaaagccatatcaaccaacttatacaaaaaataataaacattcacttccatttctaatgcatggtgctgaaaaagtccttgtatgtggaatattgttcacctttaaggaacctgctctcaagagctgatgcgggactttttttagggcagttctgttgtctctggctgttttgttcatttaattggcacctacaagtctctttgaacattaaaataaaataaagattgtggaggaatagaatacaaacacatagtaaggtgagatttgcataacagagtatagtaaacgatttgtgcctgattctttttgcattctctttgaatcatttttagcctttattctaagtccccaattattgtcatccttttcccaacaagattgtttctctccgccacggacattctggtcagggtctctgcttaaccatcttgacctcctgaacactctgtttgtcctgataacctgatttatgctcaaatgatgctcttccataggacggcttcctgctttgcccaaagagcattcaatttttcaagctgtttagggctccttcctcacccagggtctatttgaaaccttagagggaaggctattctttccaggaagagaaccctgctgggttgtaacctcaatctgtaaatccactggggtaactggggttagctcagttactccagagcttgctctctgagaactggatggtgctgctacttcccataaaggctgaataaaaagaggcatctgcaggcaggagaaagcgctatggtcattgctggaagattccttctgaccattagctatctctctgacctggtgtgagaagggtgacaaaaatcggagacttgaaaacaggccaaaaaaaaaaaaatggattcaaaagaattttaaaagaatcatgcacaagttcttaattagattcttttatccaaatccattttgtctggaaaataataccttactacgtatctgtattctattcctccataatctattttattttattttaatgttcacaagaagctggatgctagctaccaaatgagcaaatcagccacgataacagaactgcactaaaatctctcatcagatattgatacagtcaagaccctcatgagtgcctatgatacaaattcagtgtgagaggccagctttccgcaaggagaaggcaaccaaagcggtagctaatactgagcagttcctattgcccagatccatttctaggtgctgagatccagccagagaatcccacagtcctcatttttcatatgaagaaacatgtgagtgattcaccaccccaatcctcatgtatcatcagttttcaaacaaagccaagtagcctcctgtgcaaaaagctctcctaacccccagttgccttgataggtaaaagtattcttatgacagtgctagaaaaacacgggcacaagtgttccggcaaggtgactagaaggcaaggctaaagttgtcaaggtgacaaagtccctgatggtcctcttgaaagctgaacgtgccacctcatatgtatatgtgtatgtgtggatgcatatgtgtatgttgtgtgtacacacctacacatatatctacaaatgcatgtgtgtatgcatgcatgtgtgtacacgtgcatgcgcacatgtatctgtatacatgtattatgtacacagtatgcatgtgtacatgtatgtgtgtctgtgcatgtgtagatgtatacatgcatgtacacatgcatctacatatgcatgtgtatgcctaaatgtgtgtacaagtgcgtgcatatgtgcactatacatatgtgtacattacgtgtgtgtatgtttctacacgtgtatctg

SEQ ID NO: 13956 - RNA, 7656 nt, Homo sapiens
  source 1..7656: mol_type = other RNA
gctgggattacaggcatgagccacccctcctggcctgggtttaactattttattttatgacagggtctcactttgttgtccaggtaccggtgcgttctctgttcactgcaacctccacctcctgagttcaagcgatcctcccacctcagcctcctgagtagctggaactacagatgcataccaccacacccggctaatttttgtatttgttgtagagacaggttttcactgtgttgcctaggctggtctcaaactcctggtgtcaagggatccactgatctcggcctcccaaagtgctgggattacagaaatgagccaccacgtctggccctgggcttacctttcaagtcaactttgattcattgtcttccttgaaacaccacattcagtgattagtcaaataatgaacattattcttgcacaactcttttgaatctatcaattactttctactcatttagtacatattcactggggagatgctctgtgccagacactgtagtaagatcaggtaattcagaggaagtatagacaccccagacctcaaacgaagacaagataaatatggacaagggaagatccacctccacattcaccattttcagtctttctgtcatttccagctaaataacgtcttcaaaaatgtttcaaaataactaagtcactatttcaaactctttcaataatagcacccttctatacactggactactcttaattttctcattataacatgatcttgcttttcttttaatttttgtctttgctttctacctgaatttttattttgcattatgaaattgataggtccattactggatggcatggttcaattctccagtatgtctgttgatttgtgttccactaaatcttccaattactcagagaggagtgttaatgactgcaactataactggatttttctatttttacttggcgtatccaattttgtttatgagttttgaagctctgtgtcctcatatacatttgggacaatattctcctgaaaaattgacaatcataattatttaggaggcctcattattcctgaaaagtttctctgctttcaaatctactttgtctgattttatatatatacaccacagctgtctttgattaatgcttgcatgaggtatcttttcccactcttttctttcaatctgctctataacttttattcttatttataagtgtattgcaggtggctttctttagtcagcatatttatttttaacacattctgatgatctctagtttttacttaatgcatttagataatttacatataatgttattatagataagtttttagatagatctactatttaataatttattaaccttttttccctttgttttaattcttctatgttcctctgtctatcttgttttggtttatttcaatctggttgttaagtggtctagggattaccatatacatatataacttttcacagtatactaagaatcaatattttaccattcaagttgaatatagaaacttcatcaagagttagtcccattacatttacccttttatcttatgtatgtagtacatctagatacaatgacaactgcatcagataaagttacaatttttgctttcaaccatcaaacataccttaaggaactcaagagaagaataatagtctgttatgtctacccagacattttctatttctgcttttgttccttcattgatgatgttctaagtttccttctggtatcacttttcttatctcaaacctttgctaattcttttccagcagttttgctaggactgagaatgtatttatttaccttccaatgagaatgcatttatttgcctttatgtctggaagatacttttgctccacataccattctgggttgataatgtatttttcctttggtatttactgaatgttatgacatttttttctggctcctgggttcccgatgagaaatctacaatcattcatttggtattttatctttcatttccctttggctgctttcaaaattgttttgtgttttcttaattttccgcagtttgattatgatatgtcttgcaatgggtttcttttggtttatcctgcttgacatttactgaactttaaaaatctggtttatatcttttgagaaatttgatacattttcagccattaattcttcacagttttatcccacaaagacctctttgtcctcttacaataatgtgaatgtttccagattacaataatgtgaatgttagatttgttattttttatttgtccctgagcctctgttcagggacaataaaatcctcctttctttctataggtcagattctgtaggtattcttgttccgttttcaagttcattgactttttccttagtcttctgcatactgctattgagatcatccaattaagctttttatttcccctaatagttttggttaatactttttttaattcttaagtttaaattggtgtttacatattccaaatatttggtgagactttccaactttccattcacttcatgaatgctatcccgtaattctaggagcattgttataataactgctttaatgtatgtgtcagatgattttgacatatgtgtcctctcaatattgttatgcaaggattctctttgccatgtgaattaagatctccctggtttttcataatgctgaatattttggggcttgtaacctggacttctttggattatgtgatgagacactgtgtcttgttgaaatcttaaggataatattgctctttttgtttttgcaggcacacaattgccttgtatttaagctccaagtaccaaccagacttccatgtgttgttgtttcacagataactctatttgaaagccttgacactgcggatgagagatctctggagtgtgtgcaaccagtggtcagtgaggactggaaagtggaccattgtttagttcagtcctcaggctctttttaggtaagttgtttgggattagacccacttattcacagctggcaggtgcgtccacaagctcatgaacaactttatgggtttgctttctacagtatctgtccaggcacattctagttacttgacacatcctggtttcagtcctctcaccagaaagccagggctgtatttacccaggtggctctgccctgcacttttcacagttgcctcacattcaagctgtcttgctgctttttttcctcttgtggcccagtcatctagcttttcccttcttcagagatcttagtcactcttcttttccgtagtctccttaaggaactcaagggaagaataatagtctgttatgtctacccagacatgttctatttctgcttttgttccttcactgatgatgttctaagtttccttctggtatcatttttcttatctcaaatctttgctaattcttttccagcagtcttcctaagaatgagaatgtatttacttaccttccactgagaatgcatttatttgcctttatgtctggaagatacttttgctccacatagcattctgggtcgatatgtctttttcttttgttacttaccgaatgttatgacattttttctggcccctatggttcctgatgcgaaatctacaatcattcatttggtagtttctctttcatttccctttggctgctttcaaaattgttttgtattttcttagttttcagcagtttgattatgatatgccttgctatgggtttctttgggtttatcctgattgacatttactgaactttaaaaatctggtttatatcttttgacaaatttgaaccattttcagctattaattgttcaaagttttatcccacaaagaccactttgtcctcttctttccagattacaataatgtgaatgttggatttgttattttttatttgtgcctgagcctctgttcagagacaataaaatcctcctttctctctatagttcagattatgtaggtattcgtgttctgttttcaagttcattgactttttccttagtcttctgcattcgattatggagatcctccaattaagctttttatttcccctaagagttttggttaatacatttttttaattcttaagtttaaattggtgtttatgtattcgaaatatttggtgagactttccaactttccattcacttcacgaatgttatccccgattctaggagcattgttataatatctgctttaatgtatgtgtcagatgattttgacatctgtgtcctctcaatattgttattcgaggattctctttgccatgtgaattaagatctccctgttttttcataatgctgaatattgtggggcttgtaacctggacttctttggattatgtgatgagacactgtgtcttgttgaaatcttaaggataatattgctatttttgtttttgcaggcacacaattgccttgtatttaagctccaagtaccaaccagactttcatgtgttgtcgtttcaaagataactctatttgaaagccttgacactgctgttcagagatctccaaagtgtgtgcaacccagtggtcagtgaggactggaaagtgggccattgcacagttcagctctcaggctctttttaggtaagttgttcgggattagagccacttattcacagctggcaggtgcgtccacaagctcatgaacaactttatggttttgctttctacagtatctgtccaggcacattctagttacttgacacatcttggtttcagtcctctcaccagaaagctggggctgtatttaaccaggtggctctgtcctccacttttcacaattgtctcacatttaggaccaagctgcaggcagaaacagggagaaaagagcagttttatatgtcctttggtttcacagctcctcgaagaaacagaaaattaattacacagtagatctacactatactgaatgccagcaggaagctgtcaccagtcctgtattgttgctgctcctatgtcttgaaccaaagacaccgagagcagtgtcttgctctcagacactgactcgggtttgggtacctaaataataaagcttggagaatgtgggcattgatcccactacctcttgcatgctaagcaagcgctctaccacttgagctaattccccatatcagggaagctttgtttatccttagtgggtggcctggaacacaggtgatttcagggccttcagcgggaaagcagggctctactaagagcagatcttctcattgatggcgcagggcaaggtgcagtggctactcattctctgcaaagaaggaggaaaaaagggaagaaggagaaagtcacaaagggaaaactcacgctgccaaaatgtgaagtttagggtattccaggacagaaaaagacacgtcccagcaaagaagacctatctagacctgcccagctaaagtgtcactgatttttaaaaaataattaaataattaaaaatgattaaatgattgtgtgtgtattgcatgtgtgtgtgtgtgtgtttataaaagtgggatggcattatcacttgttccttgtagctgagactctctgggggttgtgagatggtccagatttctggaaggcacaaaagggattctgaattaatatctgatgaatgaatccactcatttatttgtatttgttatgtgaatgaatgttacaggaatcacctggtgtggagaaaacagatggcaagactatgtgctagggtaaagcaagagctcacgtgtttttgtttttggttttttaatttagaaaaaaaatctgcttttcatatctggttttcctatttaaagctatgtgatttaaggaaaatggtttaactcctctgagctttagtgtcatctacaaaatttggataatgatactgagggaagctgaaaagccatatcaaccaacttatacaaaaaataataaacattcacttccatttctaatgcatggtgctgaaaaagtccttgtatgtggaatattgttcacctttaaggaacctgctctcaagagctgatgcgggactttttttagggcagttctgttgtctctggctgttttgttcatttaattggcacctacaagtctctttgaacattaaaataaaataaagattgtggaggaatagaatacaaacacatagtaaggtgagatttgcataacagagtatagtaaacgatttgtgcctgattctttttgcattctctttgaatcatttttagcctttattctaagtccccaattattgtcatccttttcccaacaagattgtttctctccgccacggacattctggtcagggtctctgcttaaccatcttgacctcctgaacactctgtttgtcctgataacctgatttatgctcaaatgatgctcttccataggacggcttcctgctttgcccaaagagcattcaatttttcaagctgtttagggctccttcctcacccagggtctatttgaaaccttagagggaaggctattctttccaggaagagaaccctgctgggttgtaacctcaatctgtaaatccactggggtaactggggttagctcagttactccagagcttgctctctgagaactggatggtgctgctacttcccataaaggctgaataaaaagaggcatctgcaggcaggagaaagcgctatggtcattgctggaagattccttctgaccattagctatctctctgacctggtgtgagaagggtgacaaaaatcggagacttgaaaacaggccaaaaaaaaaaaaatggattcaaaagaattttaaaagaatcatgcacaagttcttaattagattcttttatccaaatccattttgtctggaaaataataccttactacgtatctgtattctattcctccataatctattttattttattttaatgttcacaagaagctggatgctagctaccaaatgagcaaatcagccacgataacagaactgcactaaaatctctcatcagatattgatacagtcaagaccctcatgagtgcctatgatacaaattcagtgtgagaggccagctttccgcaaggagaaggcaaccaaagcggtagctaatactgagcagttcctattgcccagatccatttctaggtgctgagatccagccagagaatcccacagtcctcatttttcatatgaagaaacatgtgagtgattcaccaccccaatcctcatgtatcatcagttttcaaacaaagccaagtagcctcctgtgcaaaaagctctcctaacccccagttgccttgataggtaaaagtattcttatgacagtgctagaaaaacacgggcacaagtgttccggcaaggtgactagaaggcaaggctaaagttgtcaaggtgacaaagtccctgatggtcctcttgaaagctgaacgtgccacctcatatgtatatgtgtatgtgtggatgcatatgtgtatgttgtgtgtacacacctacacatatatctacaaatgcatgtgtgtatgcatgcatgtgtgtacacgtgcatgcgcacatgtatctgtatacatgtattatgtacacagtatgcatgtgtacatgtatgtgtgtctgtgcatgtgtagatgtatacatgcatgtacacatgcatctacatatgcatgtgtatgcctaaatgtgtgtacaagtgcgtgcatatgtgcactatacatatgtgtacattacgtgtgtgtatgtttctacacgtgtatctg

SEQ ID NO: 13957 - RNA, 7756 nt, Homo sapiens
  source 1..7756: mol_type = other RNA
gctgggattacaggcatgagccacccctcctggcctgggtttaactattttattttatgacagggtctcactttgttgtccaggtaccggtgcgttctctgttcactgcaacctccacctcctgagttcaagcgatcctcccacctcagcctcctgagtagctggaactacagatgcataccaccacacccggctaatttttgtatttgttgtagagacaggttttcactgtgttgcctaggctggtctcaaactcctggtgtcaagggatccactgatctcggcctcccaaagtgctgggattacagaaatgagccaccacgtctggccctgggcttacctttcaagtcaactttgattcattgtcttccttgaaacaccacattcagtgattagtcaaataatgaacattattcttgcacaactcttttgaatctatcaattactttctactcatttagtacatattcactggggagatgctctgtgccagacactgtagtaagatcaggtaattcagaggaagtatagacaccccagacctcaaacgaagacaagataaatatggacaagggaagatccacctccacattcaccattttcagtctttctgtcatttccagctaaataacgtcttcaaaaatgtttcaaaataactaagtcactatttcaaactctttcaataatagcacccttctatacactggactactcttaattttctcattataacatgatcttgcttttcttttaatttttgtctttgctttctacctgaatttttattttgcattatgaaattgataggtccattactggatggcatggttcaattctccagtatgtctgttgatttgtgttccactaaatcttccaattactcagagaggagtgttaatgactgcaactataactggatttttctatttttacttggcgtatccaattttgtttatgagttttgaagctctgtgtcctcatatacatttgggacaatattctcctgaaaaattgacaatcataattatttaggaggcctcattattcctgaaaagtttctctgctttcaaatctactttgtctgattttatatatatacaccacagctgtctttgattaatgcttgcatgaggtatcttttcccactcttttctttcaatctgctctataacttttattcttatttataagtgtattgcaggtggctttctttagtcagcatatttatttttaacacattctgatgatctctagtttttacttaatgcatttagataatttacatataatgttattatagataagtttttagatagatctactatttaataatttattaaccttttttccctttgttttaattcttctatgttcctctgtctatcttgttttggtttatttcaatctggttgttaagtggtctagggattaccatatacatatataacttttcacagtatactaagaatcaatattttaccattcaagttgaatatagaaacttcatcaagagttagtcccattacatttacccttttatcttatgtatgtagtacatctagatacaatgacaactgcatcagataaagttacaatttttgctttcaaccatcaaacataccttaaggaactcaagagaagaataatagtctgttatgtctacccagacattttctatttctgcttttgttccttcattgatgatgttctaagtttccttctggtatcacttttcttatctcaaacctttgctaattcttttccagcagttttgctaggactgagaatgtatttatttaccttccaatgagaatgcatttatttgcctttatgtctggaagatacttttgctccacataccattctgggttgataatgtatttttcctttggtatttactgaatgttatgacatttttttctggctcctgggttcccgatgagaaatctacaatcattcatttggtattttatctttcatttccctttggctgctttcaaaattgttttgtgttttcttaattttccgcagtttgattatgatatgtcttgcaatgggtttcttttggtttatcctgcttgacatttactgaactttaaaaatctggtttatatcttttgagaaatttgatacattttcagccattaattcttcacagttttatcccacaaagacctctttgtcctcttacaataatgtgaatgtttccagattacaataatgtgaatgttagatttgttattttttatttgtccctgagcctctgttcagggacaataaaatcctcctttctttctataggtcagattctgtaggtattcttgttccgttttcaagttcattgactttttccttagtcttctgcatactgctattgagatcatccaattaagctttttatttcccctaatagttttggttaatactttttttaattcttaagtttaaattggtgtttacatattccaaatatttggtgagactttccaactttccattcacttcatgaatgctatcccgtaattctaggagcattgttataataactgctttaatgtatgtgtcagatgattttgacatatgtgtcctctcaatattgttatgcaaggattctctttgccatgtgaattaagatctccctggtttttcataatgctgaatattttggggcttgtaacctggacttctttggattatgtgatgagacactgtgtcttgttgaaatcttaaggataatattgctctttttgtttttgcaggcacacaattgccttgtatttaagctccaagtaccaaccagacttccatgtgttgttgtttcacagataactctatttgaaagccttgacactgcggatgagagatctctggagtgtgtgcaaccagtggtcagtgaggactggaaagtggaccattgtttagttcagtcctcaggctctttttaggtaagttgtttgggattagacccacttattcacagctggcaggtgcgtccacaagctcatgaacaactttatgggtttgctttctacagtatctgtccaggcacattctagttacttgacacatcctggtttcagtcctctcaccagaaagccagggctgtatttacccaggtggctctgccctgcacttttcacagttgcctcacattcaagctttaaggaacctgctctcaagagctgatgagggactttttttagtgcagttctgttgtcactggctgttgggctcatttagttggcaccaacaaatctctgtcttgctgctttttttcctcttgtggcccagtcatctagcttttcccttcttcagagatcttagtcactcttcttttccgtagtctccttaaggaactcaagggaagaataatagtctgttatgtctacccagacatgttctatttctgcttttgttccttcactgatgatgttctaagtttccttctggtatcatttttcttatctcaaatctttgctaattcttttccagcagtcttcctaagaatgagaatgtatttacttaccttccactgagaatgcatttatttgcctttatgtctggaagatacttttgctccacatagcattctgggtcgatatgtctttttcttttgttacttaccgaatgttatgacattttttctggcccctatggttcctgatgcgaaatctacaatcattcatttggtagtttctctttcatttccctttggctgctttcaaaattgttttgtattttcttagttttcagcagtttgattatgatatgccttgctatgggtttctttgggtttatcctgattgacatttactgaactttaaaaatctggtttatatcttttgacaaatttgaaccattttcagctattaattgttcaaagttttatcccacaaagaccactttgtcctcttctttccagattacaataatgtgaatgttggatttgttattttttatttgtgcctgagcctctgttcagagacaataaaatcctcctttctctctatagttcagattatgtaggtattcgtgttctgttttcaagttcattgactttttccttagtcttctgcattcgattatggagatcctccaattaagctttttatttcccctaagagttttggttaatacatttttttaattcttaagtttaaattggtgtttatgtattcgaaatatttggtgagactttccaactttccattcacttcacgaatgttatccccgattctaggagcattgttataatatctgctttaatgtatgtgtcagatgattttgacatctgtgtcctctcaatattgttattcgaggattctctttgccatgtgaattaagatctccctgttttttcataatgctgaatattgtggggcttgtaacctggacttctttggattatgtgatgagacactgtgtcttgttgaaatcttaaggataatattgctatttttgtttttgcaggcacacaattgccttgtatttaagctccaagtaccaaccagactttcatgtgttgtcgtttcaaagataactctatttgaaagccttgacactgctgttcagagatctccaaagtgtgtgcaacccagtggtcagtgaggactggaaagtgggccattgcacagttcagctctcaggctctttttaggtaagttgttcgggattagagccacttattcacagctggcaggtgcgtccacaagctcatgaacaactttatggttttgctttctacagtatctgtccaggcacattctagttacttgacacatcttggtttcagtcctctcaccagaaagctggggctgtatttaaccaggtggctctgtcctccacttttcacaattgtctcacatttaggaccaagctgcaggcagaaacagggagaaaagagcagttttatatgtcctttggtttcacagctcctcgaagaaacagaaaattaattacacagtagatctacactatactgaatgccagcaggaagctgtcaccagtcctgtattgttgctgctcctatgtcttgaaccaaagacaccgagagcagtgtcttgctctcagacactgactcgggtttgggtacctaaataataaagcttggagaatgtgggcattgatcccactacctcttgcatgctaagcaagcgctctaccacttgagctaattccccatatcagggaagctttgtttatccttagtgggtggcctggaacacaggtgatttcagggccttcagcgggaaagcagggctctactaagagcagatcttctcattgatggcgcagggcaaggtgcagtggctactcattctctgcaaagaaggaggaaaaaagggaagaaggagaaagtcacaaagggaaaactcacgctgccaaaatgtgaagtttagggtattccaggacagaaaaagacacgtcccagcaaagaagacctatctagacctgcccagctaaagtgtcactgatttttaaaaaataattaaataattaaaaatgattaaatgattgtgtgtgtattgcatgtgtgtgtgtgtgtgtttataaaagtgggatggcattatcacttgttccttgtagctgagactctctgggggttgtgagatggtccagatttctggaaggcacaaaagggattctgaattaatatctgatgaatgaatccactcatttatttgtatttgttatgtgaatgaatgttacaggaatcacctggtgtggagaaaacagatggcaagactatgtgctagggtaaagcaagagctcacgtgtttttgtttttggttttttaatttagaaaaaaaatctgcttttcatatctggttttcctatttaaagctatgtgatttaaggaaaatggtttaactcctctgagctttagtgtcatctacaaaatttggataatgatactgagggaagctgaaaagccatatcaaccaacttatacaaaaaataataaacattcacttccatttctaatgcatggtgctgaaaaagtccttgtatgtggaatattgttcacctttaaggaacctgctctcaagagctgatgcgggactttttttagggcagttctgttgtctctggctgttttgttcatttaattggcacctacaagtctctttgaacattaaaataaaataaagattgtggaggaatagaatacaaacacatagtaaggtgagatttgcataacagagtatagtaaacgatttgtgcctgattctttttgcattctctttgaatcatttttagcctttattctaagtccccaattattgtcatccttttcccaacaagattgtttctctccgccacggacattctggtcagggtctctgcttaaccatcttgacctcctgaacactctgtttgtcctgataacctgatttatgctcaaatgatgctcttccataggacggcttcctgctttgcccaaagagcattcaatttttcaagctgtttagggctccttcctcacccagggtctatttgaaaccttagagggaaggctattctttccaggaagagaaccctgctgggttgtaacctcaatctgtaaatccactggggtaactggggttagctcagttactccagagcttgctctctgagaactggatggtgctgctacttcccataaaggctgaataaaaagaggcatctgcaggcaggagaaagcgctatggtcattgctggaagattccttctgaccattagctatctctctgacctggtgtgagaagggtgacaaaaatcggagacttgaaaacaggccaaaaaaaaaaaaatggattcaaaagaattttaaaagaatcatgcacaagttcttaattagattcttttatccaaatccattttgtctggaaaataataccttactacgtatctgtattctattcctccataatctattttattttattttaatgttcacaagaagctggatgctagctaccaaatgagcaaatcagccacgataacagaactgcactaaaatctctcatcagatattgatacagtcaagaccctcatgagtgcctatgatacaaattcagtgtgagaggccagctttccgcaaggagaaggcaaccaaagcggtagctaatactgagcagttcctattgcccagatccatttctaggtgctgagatccagccagagaatcccacagtcctcatttttcatatgaagaaacatgtgagtgattcaccaccccaatcctcatgtatcatcagttttcaaacaaagccaagtagcctcctgtgcaaaaagctctcctaacccccagttgccttgataggtaaaagtattcttatgacagtgctagaaaaacacgggcacaagtgttccggcaaggtgactagaaggcaaggctaaagttgtcaaggtgacaaagtccctgatggtcctcttgaaagctgaacgtgccacctcatatgtatatgtgtatgtgtggatgcatatgtgtatgttgtgtgtacacacctacacatatatctacaaatgcatgtgtgtatgcatgcatgtgtgtacacgtgcatgcgcacatgtatctgtatacatgtattatgtacacagtatgcatgtgtacatgtatgtgtgtctgtgcatgtgtagatgtatacatgcatgtacacatgcatctacatatgcatgtgtatgcctaaatgtgtgtacaagtgcgtgcatatgtgcactatacatatgtgtacattacgtgtgtgtatgtttctacacgtgtatctgc

SEQ ID NO: 13958 - RNA, 1844 nt, Homo sapiens
  source 1..1844: mol_type = other RNA
gctgggattacaggcatgagccaccctgccaggcccagcgtctattgattcctatttctagaggaaatttcccctgaggcccttgatcttgaaagatgtaaataactcaactgaaaatgttacttacttattctctttggtttcaaattgcctcctttctatcaagttggctatgctctgaggaaagagaagacagacaaggaatgcacatagttctatttcagcagctcagggcgaagtgggcacatgaggggtacttgaccgtatggaggaaatggggagaaggtccagattgagttaccttgtagcacctgtgcaacaacattcgggcagctgacaggatgttcacagtatataaatagaaggtcctggatggggcatggtctggtgttttgggaatttcctggagtgacatgaaattttctgagagcatcttatatagcatatcctttgcctcctttgcaggaatcattgcaaagtcttccacttgcttctgctctatgtgtttcttctgcaaaactagacggaatattctagcacagcgagacccaaattggatcatctgccagcagagtgagatactgatcaagaacttgcttagagatgttatagccaacaggtagggatctgaagatctcattggaagacaatggctgggtgaagggagcactagaggaagtggtaatctcactcattcggagcatggttcgcacaatctcgctgcttgtctgtttgaaaagtaaactggtccatcctgttagcaactgcgctcacaatggcttggtcacggaagtgttggtggaatctgtcaaggttggcctgccaataaatcccatcatctggaatgggctccttgttatctgtagtatattttggtctcttggccttgggctccccagcagcatcttcatcagatgatctcctccttttacctttccctatcaagctgagtttaggaaccaggtacatgtccttttcattaatgacaagtgtgggggcaggtggtggtggcccagggtctgaattctcagtggtaggtaccgaagggcagcgttgtacaaagtgtgtgtctgccagtcgcacaaatgtgtttgatacttcagcatagtccatggtcttgccatcctccatggtctctgtgagccggtctgccactttcttcacaacagctgacattgtcagtttgccgttcaacagaagctcctcaacaatcagctctccagtgtcactgtacagagttttggtagtatagatgtaccggggatatctaagcattcgcaatacccggctgcactgggcttcatactccaccacaccacgtttgtgcacttgataactcaccaggttatgttggacgaggacacacagggctttcttcacctgatccagtgatgttcctgtgtcatgggcaattactcttagtggctggctgccggttcttatcagatggactccaattttttctacaatctctccaaaatgctcttgcagcaacaaagaacagagcttaatttctgcttgagtcattgtactggggagtctgagagctcagggtcagcgcaatccgggggctccaactccaattcggctgagcttcccgcgacggcttcctacggctcccgctggccttctaggccgaggtggagcccaccgccctttctaggacgcggatcgccaccgaagaagacgcggaaaagcaaaaagcgcgtgccactctaccccagagtttcggcggcttccggggacgctctttctttcttctcgctggaagactggaggaccagcgaggggctgtttgtggagccggcgggcgggccgtttgtctctccttcctgcgcctcttt

SEQ ID NO: 13959 - RNA, 1316 nt, Homo sapiens
  source 1..1316: mol_type = other RNA
gctgggattacaggcatgagccaccctgcccggccccatatttttttagctagcttcccaggtccttctgatatgtacccaagcaccatagccctcaggaaaacaaaaatatgtttattcagtaaacatatatagggtacctgccatgtgccaagagtcattctaggtgctgtggacacaacagtaaaaaaactagacaacagagtccttctgtttaaagggctgtcgttcaggactggactggacagcaggaggtgaatggcgagcgagtgagccaagcttcatctgtgtttacagccgctccccttcactcacgtgactgcctgagctccgtatcaagactcttcacattttcttgggaaatttttgtagtaggatgagataagactcagttaaaaggaagaccgccatttggtgagtgattcaaaatcttgttagttcagatttccctgcagtggagagaaagaacatggtagattaaccaagaccccgaattatctgctgcgcggcccatggagaggtgggatctaattcttcctttgagtacaggccagccttagtgattggcttgccaatggaccacaacagcagaggtgctctggcccttccgaggcaggtgtcagaagcgttgcttgctgattctgcaggggacccctggaaacactccctccggggaatccagcatctgtgtgaggagtctgaggcttccgtgacgtcaccatgctggagaggccacgtgtaggaggcagtcccagctgagcccagcctggcaggcatccgagctagggcccccaatagtgagtgcagccaccttgtatcttcccagccagctcatctgccagctgtggagcgacttccagcaacaccagtgaggagcagaaaaaattttccaaattcctgacccacaaaatcaagagatacaatagtttgtgataggtttattatatatataatatgtaatatatgacttattataaattaattgtgagattcacagtctcacaaggcagatgtggaaataagtaattacattatattgtgaaataatagatgtcatcattatataaaacttataattatgtaagttgtacataatttataatacatgtaatagaaaataggttgtagatttaagcaccaagttttagggcagattgttaagtggcagtcgctgaaacagggtgggactgcacgctgcacgcctatgatcagggtgagggtggagaccctaggaaaagtaccgctctgcagactttgtgtcttaggagtgtcctgacataccgctgggaggattacctcatccattccttcttttt

SEQ ID NO: 13960 - RNA, 1155 nt, Homo sapiens
  source 1..1155: mol_type = other RNA
gctgggattacaggcatgagccaccctgcccgggctccacaatattcttaaccacttgtattaggtctctttccattcaaagttatggaaacccaggtcacactccttaagtgggtgaaaagtaaaaagtgcagaagtatggggattgaggatcagacaacataaacaaggttctgtctctctcttggcatccagctctcggcagactactacacactgtgcatgatataccaagactaaaagactcataacctacccgcagaaagagtgcatcttccatagtagctctgcaaaaagatccaaaagaaactgttaatggcctggcttaagtcaaattgtgtccggaattggtgggttcttcgtctcactgacttcaagtatgaagccgaccctcacggtcagtgttacagctcttaagatggcgcctctggagtttgttccttctgatgttcggatgtgttcggagtttcttccttctggtgggatcgtggtctcgctggctcaggagtgaagctgcagaccttcgcagtgagtgttacagctcttaaggcggcgcgtctggagttgttcctttctcccggtgggttcctggtcttgctggcttcaagagtgaagctgcagaccatctctttcatctgccctctgtagatagcgtgcaatagtatacaactgttttcctttacagatttccactggaggtctcagcaaagggttgtcatcaaaatttatctccttcagtgaaaaaatattgtagatagcactaggtagagctgtcagattatttccactcaggtttagttgctgcagatcatttaaagatagcaaagatggtggaagataacttatttgattattgtatgcatgtaaactaaccaaatttctcaattctcctatatttcttggaatctctctgattgcattatttgagatatcaagttctttaagttgagtcatattagatagctctcctggaagtcttgttagagggctgctgaagtaagacacacccttcgcttcacctgtggcctcccgcggcggctgcggctccttcgcaggaccggtagggggcgcgcgcggttgagtccagcaattgcgaggacctccgcaggcgcagcccagcactgacgcctctccgggccgtggctcctctttccc

SEQ ID NO: 13961 - RNA, 1132 nt, Homo sapiens
  source 1..1132: mol_type = other RNA
gctgggattacaggcatgagccaccctgcccgggctccacaatattcttaaccacttgtattaggtctctttccattcaaagttatggaaacccaggtcacactccttaagtgggtgaaaagtaaaaagtgcagaagtatggggattgaggatcagacaacataaacaaggttctgtctctctcttggcatccagctctcggcagactactacacactgtgcatgatataccaagactaaaagactcataacctacccgcagaaagagtgcatcttccatagtagctctgcaaaaagatccaaaagaaactgttaatggcctggcttaagtcaaattgtgtccggaattggtgggttcttcgtctcactgacttcaagtatgaagccgaccctcacggtcagtgttacagctcttaagatggcgcctctggagtttgttccttctgatgttcggatgtgttcggagtttcttccttctggtgggatcgtggtctcgctggctcaggagtgaagctgcagaccttcgcagtgagtgttacagctcttaaggcggcgcgtctggagttgttcctttctcccggtgggttcctggtcttgctggcttcaagagtgaagctgcagaccatctctttcatctgccctctgtagatagcgtgcaatagtatacaactgttttcctttacagatttccactggaggtctcagcaaagggttgtcatcaaaatttatctccttcagtgaaaaaatattgtagatagcactaggtagagctgtcagattatttccactcaggtttagttgctgcagatcatttaaagatagcaaagatggtggaagataacttatttgattattgtatgcatgtaaactaaccaaatttctcaattctcctatatttcttggaatctctctgattgcattatttgagatatcaagttctttaagttgagtcatattagatagctctcctggaagtcttgttagccttcgcttcacctgtggcctcccgcggcggctgcggctccttcgcaggaccggtagggggcgcgcgcggttgagtccagcaattgcgaggacctccgcaggcgcagcccagcactgacgcctctccgggccgtggctcctctttccc

SEQ ID NO: 13962 - RNA, 1120 nt, Homo sapiens
  source 1..1120: mol_type = other RNA
gctgggattacaggcatgagccaccctgcccgggctccacaatattcttaaccacttgtattaggtctctttccattcaaagttatggaaacccaggtcacactccttaagtgggtgaaaagtaaaaagtgcagaagtatggggattgaggatcagacaacataaacaaggttctgtctctctcttggcatccagctctcggcagactactacacactgtgcatgatataccaagactaaaagactcataacctacccgcagaaagagtgcatcttccatagtagctctgcaaaaagatccaaaagaaactgttaatggcctggcttaagtcaaattgtgtccggaattggtgggttcttcgtctcactgacttcaagtatgaagccgaccctcacggtcagtgttacagctcttaagatggcgcctctggagtttgttccttctgatgttcggatgtgttcggagtttcttccttctggtgggatcgtggtctcgctggctcaggagtgaagctgcagaccttcgcagtgagtgttacagctcttaaggcggcgcgtctggagttgttcctttctcccggtgggttcctggtcttgctggcttcaagagtgaagctgcagaccatctctttcatctgccctctgtagatagcgtgcaatagtatacaactgttttcctttacagatttccactggaggtctcagcaaagggttgtcatcaaaatttatctccttcagtgaaaaaatattgtagatagcactaggtagagctgtcagattatttccactcaggtttagttgctgcagatcatttaaagatagcaaagatggtggaagataacttatttgattattgtatgcatgtaaactaaccaaatttctcaattctcctatatttcttggaatctctctgattgcattatttgagatatcaagttctttaagttgagtcatattagatagctctcctggaagtcttgttagctgtggcctcccgcggcggctgcggctccttcgcaggaccggtagggggcgcgcgcggttgagtccagcaattgcgaggacctccgcaggcgcagcccagcactgacgcctctccgggccgtggctcctctttccc

SEQ ID NO: 13963 - RNA, 2903 nt, Homo sapiens
  source 1..2903: mol_type = other RNA
gctgggattacaggcatgagccaccctgtgctcttatacatcataccactaacagctactttttcagtttattataaagacggtgtcttgctctgttgcccaggctgtcatttgtcgaaggatcacagaagttggagttctgggctttttggctctgactcacctaggtagagccacagcctcaggatcacagttctgtctgaacacttatggagggagcagtgatcagctcagcaggattgtcaattagccttgtaagctaaactccagtgctgtgtccaccaagagctcaacaagcttcgtgctacagatcaccaccaggtggcacacgtttaatgatcatgcccatccagggtggcgggaacctgctactgccaagctcaggagttattttggcctcattctgggctgacaaaagctacattattaacctcaaactataactggatttttctttcttgcttttagtgtatttccctcattgattaagtactatattgttaggagataaaaactttgaaggctttagaaataataaactactaatgttgccaaaatttcatcccagtaaggaataggaaaaaaaaaaagctgagctctgaatacttcgtcttcatgaaaaagttgcttctgggcgtcaggtctggcgccaggcaaaagagtgaaacaggttaagtgtggcttgtacttgccatctttctccctttgctgtctgtcttctgatttcacactcctccctaatttcaaataatacccttgttaaatttttttaaaaggtttaaagcccgttttcaatgtttcgtatagaatccactgtaggtcattgtttttcatgtaacttatgtgcttccacaatgcttgatggaggccttagccttctccaaccccaccctgaaatctcaaacagtcatcccggtgggcagtccaggaggagattggtaccagctctcccattctccaagtacattgaccacagtgtagcagaatgcagctctctggaaagaaagggagaaggaaggaagaaagggaaggagagagggagggaaggagggagagaggaagggaggaagaaagggagggagggaggaaggggaatgaaggaaagaaaaaggaaatcgataatccaagacattttatatacatatatggacaattcttcacaaagtcagatcttcccatggtgccctaatatcttccagggtcacaccaggactattacacaaagtcatttacaaccactgggtaggaagaaatcttttgcacctagatctttggctggtgcagcattttacactttcagtacaatcagttgtgtttttctccatcaggtttatggtcttctcccagtcagtataccccgtagctacccctccaaattcccctctgatctggacagggatttctttgatctcctaaacccactgttccattgtaagcgctcaggtcaggaggcctctcctcttttgtacctgtaggggatccaggcacaggaggtggagggagtggaagatgggagtggaagtcttcctcatatcctttcatagggggctaggtaccctattctcgtgtttgtgtgtctcctctgagctacagtcacagaggtcactttgctttgcttggaaatgagttgaaaaaaacctcctctcgatctggcatccttcctattgttccaacaaaggtttgcttgttgggaaagcaccccagttgtccacgagtttactctcatttgaccctggggaaatattcaagtaagttcagatcaaccagaccatctcttttctgtttgttaaacttgcggtgctgaaagcataaaggaacctaccttaagtcaccaagttagagctccaatccttgctgtaacccaaaaaaactctgcttctttttatttttttcttcctcttttctataggcctctaatcacatcactcttacccagctagtcccccttcctcttcctcccatgattctctatctctcctctccaccccacccttctctgacgtctcccttcttcccttccttacttctgaaaaagggaaaaaaaagaaaaaaggaggtacattgcaagatggagaagagagggatggaagggtagaaaaagtgctttgtaaaattccagggagtagcaagccaggcctggtcagtagctgtgttaggccgttctcacattgctataaagaatagctgagactgggtaatttgtaaagtaaagaggtttaattggatcacggttctgcaggctgtacaggaagcacgatgctggcatctgctcagcctctgaggaggcctcaggaaacttacaattatggtggaaggcgaaggggaagcaggcatgtcacagggcgcagcaggagcaagacagagagacgggaggcgctacgcacttttaaacagccagaattcatgagaactcactcaccatcactatcacttggtgggacagtagcaaaagggatggtgctaaaccattcacgagaaattcaccctcatgatacaatcacctctcaccaagcccacttccaacactgggggttacatttcagtatgagagttgggcagggacacacatccaaactgtattaatagcctacccagacaagactgtcctggcccagtattcctcttagaaactgaagaaaaggaaaaaagaaaccctctgataccctacaactccctgagctttttagttgccaactttaaacaaattttcctacttacctaaatagcagtctcctactggtagctgagaatggtcttgtagatgccacctcagtgctgcatctacaacattgtgttcagtatgcttcctttagctgagaattattataactttagaagctgagaatgattttcttgaggatcagtgccattgtgttggtcctctccctgccttactgaccctc

SEQ ID NO: 13964 - RNA, 2945 nt, Homo sapiens
  source 1..2945: mol_type = other RNA
gctgggattacaggcatgagccaccgaacccagccagcatcaagagttttaaaattaaggacataacgccatttcacactttaaatagactatagtgtagtgtaaacatagcttctttttttaaatagagacaggatctccctatatgcccaggttgatctcacaattcctgggctcaagtgaccctcccgcctccgtctcctaaagtactgggattataggcatgagccatcacacccagccaatataacttcatattcacaaggaaacaaaacaatttgtgtgactcactttgtagcaatatctgctttattgtggtggtctcgaatcaaatctacaatatctttgaggtatggctgtactttctaagcatttcctgagtcagcctactttttctccatttttattgtcactattctatctattttttgttttgttttgttttgttttcttgttgttgtttggaaacaggaacttgctgtgtcacccaggctggagtgcagtagcacgatcatagctcacagcagcctcgatctcctatgttgaaaccatcctcctgcctcaggctcctgagtagctgagactacgggtgcatgctaccacacctggctcatttttaaaaagatgtttttagagatggggtcgcatgatgttgcccaggctgatctggaactcctggcctcaaacaattattccacctcagcctcctgagtagctagggtcgatccattgttgaagagtacatggatgttattttgcagactgtcaacctgaatttgtatttgcttgacattgcctaattattagtttcagtttcagcttacccactttttgtctgcaacatgcagaagagacagtgccctttttagtgtatcatatcaggaatcatctcacattggtttgtgccattactggtgcagtgactttcagccacttgggtaaggtggagttggccatatgtctccactgcaaaattactgattttccttttgtaattaataagtgtgtgtgtgaagattctttgagatgaggtatatatctcactcttcatcaaactataagttttttaagtaaaagaaaatttattatgaaactaaaggaataaaagaatgaccactccataggcagagaaacgtcactttaaggttttgacgtcaattgatttttgtccaaatcaataattactgcaatgattgaaaaatgattattactaagtttgttttcattgtctcaaggtctgctgaactctggatccaggctgtgtcaacagggtagtgtggtgcctcctgtacctgtcttggcctcctacagtcctttttacttattttgttttttagaatagagacagggtcttactatgttgctcagactggtttcaaactcctaggctcaagcaatcttccagcctcagcctcctaaagtgctgggattacaggcatgagccaccacacccggccaagttctttaccatcttcagaaggcttagcttgcacttttggaagaagaatagactcccaggaagactgtgagagagatttggggcccaaattgatattatcaaatacactgaacttgattgtattcaccatgttctggctcttgagaaatgagagtgctagtgaggctggtgccactttgtgtatcttctgtaccttgaagtccctcagaaaccttgcccctggtcttctctggtcttctcattctaaggacataacaggttctctttttctctggagatgaaatctagatcttcgattttggaaccaaatttggactcttgactctgaagcaccaatttcttcagcaagttgttctctggaatcaatcccagggtatgggtttttcataaatgcatggatgactgtgtgtaattgaaaggtgctataggtggtacaacaccatctggcttctctattttgaaactccacaccaggttaatcttgtccatggctgtggcttaaatctaaagtcaggttctggtgttttctggaatccatgcctagctctttgattctgaaaccaaatctggattctggactcttctgcattgattgctaaagcaagtttttgtttggtagcataacctgggtaaggtttttgagtgaaggtattgatgaggattttcaattgatcttctgtgaatttggtgcaattgcacctatgatttgttgctaccatcttgtgtgaagaggggtcttcaactatgcagaaagagagttctggaggctgagctactgtctgggagactgcttacagctcattttttaaaaagaaaggtcacatataatacaatataaaattcacaaatctaaagcttatggttttctgggttttgacaaatgaaaactcctgtgcaacttcaagccttaccaggatatggatgagggtttctacccaaaagcaccagtattctaacaaacaactttacgttttttgaattgtccagtgcctgtgaggattccttactccaagtttatgacaaacatattcagaaggcatagtctacaattagtgtttgggtaagtattttcatcaattgtctgattatttgctgtgaatttgaagtatgctgattcttatgtaattgtcttctgagaaacattgtgccatttttcttgtggaaaccacctttatcttgtttcctgcaaaatcatggaggtttgggaagttcctttagacccattctcgtatggaggtttgttttcttcttttttctttcctgggcgtggtggcgggtgcctgtaatcccagctactcaggaggctgaggcaggagaatggcgtgaacccaggaagcagagcttgcagtgagctgagatcatgccactgcactccagcctgggcaatacagcgagacgcggagacctgcctcctactccaccatcacatggaacccaccactgcttctccgaagctcgctctgaccacgccgctgctgctgcaggg

SEQ ID NO: 13965 - RNA, 7647 nt, Homo sapiens
  source 1..7647: mol_type = other RNA
gctgggattacaggcatgagccaccgagcccggcctatgtttatatatcttgcactacagccagtgtgtgtagctcaaggacttgcctccactgggggtgagggcactgggggagaaaactgagcagccacgtgatgaacatggtgctcctttgtggtggcataagtttcagtaaagattaaacatatcatttttatattaaaagttttattataaagaatgcaaaattcacttacattttaaagacagaacacacttcatgtcagtggtaggctgattctgattttgctctcagaaccccttcccccttcatcatgcccctctgctttagggttacgctagtggaaaaatttgagcagcaaactctaggtatgtcactttgtccctatttggtcactctacacattcttataggttctcttttataagtacatagtcttgaataaacaaagaggaaagatggtctaataaatatatagtatggtgaatactttaaggtaaccagtagtcaacactaactttgtttccaactagaattaaattcatgctgtgcaaggagtcagacaatgagcaattctcatcttactatttatacctctatggcttagggtaagatgctctgagggacaaatgtgaataagatttccttagatcttgtgctttggctccccaagtacaaggaaacctgaaatagaatgttatgtcaattgcccattcattttggttagtacgactctttcctcatcagtttctagaacaatctcagatgacaagtgaattgtaaaaggccgtaataaattaacatatagcagtatgcagacagatcaaaacaggttatgaaatagatttaaaattacttcctacaataagtcttaaatataatgacaacattaacaaaataaccaaaggtccataggcaaatgtagtttatgactaagcttaaagcattctgaatgaatacagttgagatttcttatcagtgaggtaacagggcaatagtccttcacagtaacaaaatgtgcaagggtgcctaggaaaagtgggaggtagagagaaaaaggcataaaattaaatgtatccaagtgaagtttggatttttcaagcatcacaaatatcaatggaaaatgtggaaaaaagtactgatagcagcagctcatagaacaacttatccattaaactacagctaatatccctgttgcatcaattccagaagcaacttgcttaagaaatgggaggtctatttcctatataaagacattccaaagtatccaatctcttagaacctctccatctgctaacgtatctacatcaaaataacaacatatatattcaaaacgaaaacctcaaataacctaagccactatacattcttcaagatgaacaaaattttgttcaagtctcacttaatttgccaggttaaattaaaaataacagtgaagcaggaaaattattcattgcacttatgcatcagttactcaaaacacacaaaaattgttttgtgagctaaattcttctagatatggagtgaaacccaaatgttacttttagtgccctttatgacatttttgttctaacctgagtttttaaaaaaaatgtgctggaaagaaggacccttaaaaagtcatctgtatatctcttaatttttaaaatttttattcccttaaaaataaaaaaaagattttgaatagaagatattatgaagatttctcaagaagttcctaaatcttaaactttccatgctgtctttaaaaaaaagatccttattccctctggttctgtcttcactagagatggagaacactatggcatagtatttcttactttgaacccttcaataaaagactcaataaagctttattagcaaacttagcaaactatctcaacagctttctcctctccagagtcaaacaatctttattccttgaactttttctcagaagtcttattttctaatctacattttcttcctttttatttctgctctacctcttcctgagttctcacatgattctgatacaacatcctagcaggaactgaatccgtaaaagggatactttttctcacctcctaaaccttggcctcattttagtgatcacaataaaggaaaatggtaggtgcatactcatcataacaacaaataaacacaagtaaacaggtgggacacagtttattccctactgttatggtgttacatttgcccttcacgagaagcatttcccgtgtctctttatattgtttgcttatttctactgtttatttccaatgtatgctttgatcttgccctactaattctctccttttctccaaagctttagaaaattccagttttgactttcatgctcaatgagaatgcaatcattttcacaatattgttcaaaaagaaaaagataaacattgtagtgcccgaggctgagacctcctagccagcacttctgtctctcctgaccagcttgggctatcactgaatttatcctgttaggcaaatgtgcacctactacatcaagttcatgttaagtatcatgctcagacagactcatgacaggctagaataaaataattccctcaatcgatacacttcaggaacatttgtaaaattttgttaacttgagagaagaacacttcaataacttttcaccttaagatgacttaaatgttgcattatattaaagcactcaaataaaactgttttcttcataatagaatgacagtcatgacatggctttagtaactatgaatgagccgttgattcattttagcttcatttttgtttatcagtcactgaaacacagaactaaaccaaatatacctgtttttcatatatacaacattataccactttgcagaatatatgccatttcctaaattacaatctacattcttaaaagcatataaaacaaaagatgttttacacattttaaaaataaaacaaaaattctacacatatcttctccagtgcaaagcctttgaaaacaaactcattgagaaaaatggtgctctacatttagctagctgtctattatctacagtcatacagtcatataagatccaacaataagaaagtaaggaaggaacaaattaacaatagtggcaatacaatagttggacaattaggtttggattatatgagctcaaccaaatgttagctgacagctgcaacaaacgaaaccatgatttaaggaacattctaatcagttcaaactttatattattattttatatgaaataaattctctaattacagtgctatctcccataagcaatttgtttaggtcttgttattgttatctcctaactataccccatatgtattctgagaactatgtaggacaagatacattttaagaagattaaacacagcatttctttttctctctctctctctttttttttttttttttgagataaggtctcactctgtcatccaggcttcagtgcggcagtgtgatcatagttctgtaacttaaactcctggcctcaagcaatcctcctgcctcagcctcccaaagcgctggtattacagatgtgagccaccaagcccagcctaaacagcatttctctattaaaccttttcagaagactgcatgattagccaaaagtgactttttttttttttgagatggagtctccctctgttgcccaggctggagtgtagtggcgtgatttcggctcactgcaatctcagcctcctaggttcaagcaattctcctgcctcagcctcccgagtagctgggactacaggtgcccaccaccacacccggctaatttttgtatttttagtagagacagggtttcaccatattggccaggctagtctcaaactcctgacattgtgatccacctgcctcagcctcccaaagtgctgggattacaggcgtgagccactgcgcccagcccaaaagtgactttttgtaaaaaattattttctacactaaaagaagataaataatagtcatgcaatcagaaattctacagaagtcagcaagatgttagaataaactggacctctgttttaaaacatgtagttttagtatttcataatacttaaaatttggatgttttattcttagtaaaattaacattacttcataaaataaaagaataaatctacttacaaaaatgtaattcaaaagttagactgtcaaataaattcagagctcctttctcagttcagatttttttctgtaataaaaggtttgataaatgacacaattctaatatgaagatccttaactacattaagcttgcttttattaagatctttatttatattcctaagattttaaaatcagcaaactcacttgatatagaggaagcacctacagattttggaagattttccttagctatctgcaaattgactgattaaattatggtaaatgcaggaacactgttttttctgttcacaccagaccctgagaaggcactgagaaatttgataagaacaaagccaataggagtgttgccactattgttttatgttcagtaaacatcagaattttaaatacatacagtaaatttatactgcaccaagggcacctgaaacagacatgccaaaaccacacactgtaacatctgttctaaactacagaaatgctaaatatcctatttcaaatactctaatttgtaaattaatacctgtgatgtcacaatgacactttttcataacaatcaaggaaagtaccattttcttgccaattttatggactaatttccttaactaaccctacaattatataacatttacctgtctttttttttttcttttaccatgctatacacaattacgagatacagaactaggcttaatcacactataataagaaaactcacttttgaattgtgatgtttctgttaacggaaggacaatacgttactataatacttttagtgtaataacttttgtttgaattatgaaaaaatttgaatcatttccctctagaccatttcatttcaaacttatactttgtttagtctagccagttgaccaaaaagaaagaaaataaaaggaaaaagatactcggccagatgagatagagagagaatgctaacacaaggttcaatgtatgcagttctcggttgctctgttccatatgcccacacagtgtcatgacatattggtgtacccctaaacagaacgccagatcagtccattcttactaggctgaagaaaattctctatcagagcatcaatgagtttcttcagttcttcctccagtaaagcagtgtcactctggtcaggtgacgcacacatctctgcataatactttatctttggttctgttccacttgtccgaagggtagcaacacagccattttgaaaagtaaatgtaatcatttggctgtttttactcacaggcagcactgatttcttattaggctggctactgtcatatccagtggtaacgtcccgtacatgcaatatagcaaatgttccacaaaattttggatattcttttggagaatcaaaattacgaagcctttcaaatatacttttgatggtaggtggttcataacacaagaaataggaagtttttgaaatatgataaccatatttttcataaaccttaaccagttgctgtttcaatgttatattcatggtttccaggtaagatgccatctcagcaaccacaacagctgcactcaccccatctttatccaaaactgaagttccacagagaaaaccaatagactcttcaaatgcaaaaaggacttctttcccattttccaggaggtctattatcctacttccaatccatttaaaacctggtaatgtttcttcaaaatgaaatccttctttaagtgcaattgccttcagaattttagaagagactgtggtggctaacatataaacgttcttcacatcagcatttcttgatttatttttcttccagcaatcaaacatccaccatccaaacaaagctgccaactcattccctgtgaaaactttccaacaaccattctcctgaagttctgctgctgccagtctgtctgcatcaggatctgtggctagcactacccgggcattttctttctctgccagtctcaaggaaagttccagcacagattctccttcttcaggatttggacatttaacggtagaaaagtctggatcaggatctttttgttctggtactggaattggaggcttaaaaccaaacactttaaaagccaactgcacatagtcatgtccgaccccatgaaaagatgtgtgcacaaatttcaaggtggtcttcgagtttaactccctgtaaaaacagatctttttcagatcttccatgtatctcctgcaaatgtcctgcagagggtctctcttcagcgggctggtatccactaaattatcattccaggaaccattccagggttccacacattcttctatacattttagaatttctttatcatgaggagatgtgatctgagcaccagtttcccagtaaaccttgtatccattgtcttccttgcggttgtgagaggcagtaatcatcacacctgcaactgctttgagcttctgaactgcatatggtacaaaaggtgtaggaacatatcttgaaaaaaggtacacaggaacatctttggccagcaagactgcagcagtgagtttagcaagcctctggctgctgcagctgctagttacttgaccccgagtgtcatacccaaccacaaagcctctctgcttgaagtctgagaaacatctctcaaggtatttgtacatcccctgtgttgactgtattactgtaaggtcattaatatagcaaaaccctgcccccatggcagaacgaagtcctgcagtcccaaaagtcattcggcaacaaagacgatctcgcagctccttgttcatcccattccgtaacaggttttcaatctgctcttttgttttgggattctgtaaaaaacaggaatcatgttctactcttcttcctgggcaccatgccagcctcccttggagcttatcccagcggagccactgcccgatggccgtgtccagctgagggtccccggtgtggtagggggcgtggagcaggttggagttcagatccccctctgtgttttcagccatggcgaccagacaggcgtacgggccgggggccggcgaagacactgagttggggtggggggtggcttggggttcgctcaccagggtccaggcgtccccacctcactgaagggcatcggagaccaaccgcagggtgttcgtaacagctcctgccgcggcgtcagggaaccgggagagagggggtttatggccgcctgctccccagcggaccaggtccgggtctctgggcgaagtgactgaggcggtcgcgccgcgagagaacaacagtcccagatgtctgggtcctggctccgccgccgccgccgccgcccgccccgcctacggccccgccccgcgccttaggccccgccccttcccgcccttgctgatttaagtccccgaagttctagactggagcccgggagcgcgctccccacgcctccgaagtagtgggggtttacagcccgtccgggtggtgaggcaatagtgcacggttctttttattttttaatttgccaagggtctcctttcctcgatctgctctcacggctaccactagcaagctgcctttgcgcttgccctgcaggtccccagcgcgcgcgcaggcccccagt

SEQ ID NO: 13966 - RNA, 7266 nt, Homo sapiens
  source 1..7266: mol_type = other RNA
gctgggattacaggcatgagccaccgagcccggcctatgtttatatatcttgcactacagccagtgtgtgtagctcaaggacttgcctccactgggggtgagggcactgggggagaaaactgagcagccacgtgatgaacatggtgctcctttgtggtggcataagtttcagtaaagattaaacatatcatttttatattaaaagttttattataaagaatgcaaaattcacttacattttaaagacagaacacacttcatgtcagtggtaggctgattctgattttgctctcagaaccccttcccccttcatcatgcccctctgctttagggttacgctagtggaaaaatttgagcagcaaactctaggtatgtcactttgtccctatttggtcactctacacattcttataggttctcttttataagtacatagtcttgaataaacaaagaggaaagatggtctaataaatatatagtatggtgaatactttaaggtaaccagtagtcaacactaactttgtttccaactagaattaaattcatgctgtgcaaggagtcagacaatgagcaattctcatcttactatttatacctctatggcttagggtaagatgctctgagggacaaatgtgaataagatttccttagatcttgtgctttggctccccaagtacaaggaaacctgaaatagaatgttatgtcaattgcccattcattttggttagtacgactctttcctcatcagtttctagaacaatctcagatgacaagtgaattgtaaaaggccgtaataaattaacatatagcagtatgcagacagatcaaaacaggttatgaaatagatttaaaattacttcctacaataagtcttaaatataatgacaacattaacaaaataaccaaaggtccataggcaaatgtagtttatgactaagcttaaagcattctgaatgaatacagttgagatttcttatcagtgaggtaacagggcaatagtccttcacagtaacaaaatgtgcaagggtgcctaggaaaagtgggaggtagagagaaaaaggcataaaattaaatgtatccaagtgaagtttggatttttcaagcatcacaaatatcaatggaaaatgtggaaaaaagtactgatagcagcagctcatagaacaacttatccattaaactacagctaatatccctgttgcatcaattccagaagcaacttgcttaagaaatgggaggtctatttcctatataaagacattccaaagtatccaatctcttagaacctctccatctgctaacgtatctacatcaaaataacaacatatatattcaaaacgaaaacctcaaataacctaagccactatacattcttcaagatgaacaaaattttgttcaagtctcacttaatttgccaggttaaattaaaaataacagtgaagcaggaaaattattcattgcacttatgcatcagttactcaaaacacacaaaaattgttttgtgagctaaattcttctagatatggagtgaaacccaaatgttacttttagtgccctttatgacatttttgttctaacctgagtttttaaaaaaaatgtgctggaaagaaggacccttaaaaagtcatctgtatatctcttaatttttaaaatttttattcccttaaaaataaaaaaaagattttgaatagaagatattatgaagatttctcaagaagttcctaaatcttaaactttccatgctgtctttaaaaaaaagatccttattccctctggttctgtcttcactagagatggagaacactatggcatagtatttcttactttgaacccttcaataaaagactcaataaagctttattagcaaacttagcaaactatctcaacagctttctcctctccagagtcaaacaatctttattccttgaactttttctcagaagtcttattttctaatctacattttcttcctttttatttctgctctacctcttcctgagttctcacatgattctgatacaacatcctagcaggaactgaatccgtaaaagggatactttttctcacctcctaaaccttggcctcattttagtgatcacaataaaggaaaatggtaggtgcatactcatcataacaacaaataaacacaagtaaacaggtgggacacagtttattccctactgttatggtgttacatttgcccttcacgagaagcatttcccgtgtctctttatattgtttgcttatttctactgtttatttccaatgtatgctttgatcttgccctactaattctctccttttctccaaagctttagaaaattccagttttgactttcatgctcaatgagaatgcaatcattttcacaatattgttcaaaaagaaaaagataaacattgtagtgcccgaggctgagacctcctagccagcacttctgtctctcctgaccagcttgggctatcactgaatttatcctgttaggcaaatgtgcacctactacatcaagttcatgttaagtatcatgctcagacagactcatgacaggctagaataaaataattccctcaatcgatacacttcaggaacatttgtaaaattttgttaacttgagagaagaacacttcaataacttttcaccttaagatgacttaaatgttgcattatattaaagcactcaaataaaactgttttcttcataatagaatgacagtcatgacatggctttagtaactatgaatgagccgttgattcattttagcttcatttttgtttatcagtcactgaaacacagaactaaaccaaatatacctgtttttcatatatacaacattataccactttgcagaatatatgccatttcctaaattacaatctacattcttaaaagcatataaaacaaaagatgttttacacattttaaaaataaaacaaaaattctacacatatcttctccagtgcaaagcctttgaaaacaaactcattgagaaaaatggtgctctacatttagctagctgtctattatctacagtcatacagtcatataagatccaacaataagaaagtaaggaaggaacaaattaacaatagtggcaatacaatagttggacaattaggtttggattatatgagctcaaccaaatgttagctgacagctgcaacaaacgaaaccatgatttaaggaacattctaatcagttcaaactttatattattattttatatgaaataaattctctaattacagtgctatctcccataagcaatttgtttaggtcttgttattgttatctcctaactataccccatatgtattctgagaactatgtaggacaagatacattttaagaagattaaacacagcatttctttttctctctctctctctttttttttttttttttgagataaggtctcactctgtcatccaggcttcagtgcggcagtgtgatcatagttctgtaacttaaactcctggcctcaagcaatcctcctgcctcagcctcccaaagcgctggtattacagatgtgagccaccaagcccagcctaaacagcatttctctattaaaccttttcagaagactgcatgattagccaaaagtgactttttttttttttgagatggagtctccctctgttgcccaggctggagtgtagtggcgtgatttcggctcactgcaatctcagcctcctaggttcaagcaattctcctgcctcagcctcccgagtagctgggactacaggtgcccaccaccacacccggctaatttttgtatttttagtagagacagggtttcaccatattggccaggctagtctcaaactcctgacattgtgatccacctgcctcagcctcccaaagtgctgggattacaggcgtgagccactgcgcccagcccaaaagtgactttttgtaaaaaattattttctacactaaaagaagataaataatagtcatgcaatcagaaattctacagaagtcagcaagatgttagaataaactggacctctgttttaaaacatgtagttttagtatttcataatacttaaaatttggatgttttattcttagtaaaattaacattacttcataaaataaaagaataaatctacttacaaaaatgtaattcaaaagttagactgtcaaataaattcagagctcctttctcagttcagatttttttctgtaataaaaggtttgataaatgacacaattctaatatgaagatccttaactacattaagcttgcttttattaagatctttatttatattcctaagattttaaaatcagcaaactcacttgatatagaggaagcacctacagattttggaagattttccttagctatctgcaaattgactgattaaattatggtaaatgcaggaacactgttttttctgttcacaccagaccctgagaaggcactgagaaatttgataagaacaaagccaataggagtgttgccactattgttttatgttcagtaaacatcagaattttaaatacatacagtaaatttatactgcaccaagggcacctgaaacagacatgccaaaaccacacactgtaacatctgttctaaactacagaaatgctaaatatcctatttcaaatactctaatttgtaaattaatacctgtgatgtcacaatgacactttttcataacaatcaaggaaagtaccattttcttgccaattttatggactaatttccttaactaaccctacaattatataacatttacctgtctttttttttttcttttaccatgctatacacaattacgagatacagaactaggcttaatcacactataataagaaaactcacttttgaattgtgatgtttctgttaacggaaggacaatacgttactataatacttttagtgtaataacttttgtttgaattatgaaaaaatttgaatcatttccctctagaccatttcatttcaaacttatactttgtttagtctagccagttgaccaaaaagaaagaaaataaaaggaaaaagatactcggccagatgagatagagagagaatgctaacacaaggttcaatgtatgcagttctcggttgctctgttccatatgcccacacagtgtcatgacatattggtgtacccctaaacagaacgccagatcagtccattcttactaggctgaagaaaattctctatcagagcatcaatgagtttcttcagttcttcctccagtaaagcagtgtcactctggtcaggtgacgcacacatctctgcataatactttatctttggttctgttccacttgtccgaagggtagcaacacagccattttgaaaagtaaatgtaatcatttggctgtttttactcacaggcagcactgatttcttattaggctggctactgtcatatccagtggtaacgtcccgtacatgcaatatagcaaatgttccacaaaattttggatattcttttggagaatcaaaattacgaagcctttcaaatatacttttgatggtaggtggttcataacacaagaaataggaagtttttgaaatatgataaccatatttttcataaaccttaaccagttgctgtttcaatgttatattcatggtttccaggtaagatgccatctcagcaaccacaacagctgcactcaccccatctttatccaaaactgaagttccacagagaaaaccaatagactcttcaaatgcaaaaaggacttctttcccattttccaggaggtctattatcctacttccaatccatttaaaacctggtaatgtttcttcaaaatgaaatccttctttaagtgcaattgccttcagaattttagaagagactgtggtggctaacatataaacgttcttcacatcagcatttcttgatttatttttcttccagcaatcaaacatccaccatccaaacaaagctgccaactcattccctgtgaaaactttccaacaaccattctcctgaagttctgctgctgccagtctgtctgcatcaggatctgtggctagcactacccgggcattttctttctctgccagtctcaaggaaagttccagcacagattctccttcttcaggatttggacatttaacggtagaaaagtctggatcaggatctttttgttctggtactggaattggaggcttaaaaccaaacactttaaaagccaactgcacatagtcatgtccgaccccatgaaaagatgtgtgcacaaatttcaaggtggtcttcgagtttaactccctgtaaaaacagatctttttcagatcttccatgtatctcctgcaaatgtcctgcagagggtctctcttcagcgggctggtatccactaaattatcattccaggaaccattccagggttccacacattcttctatacattttagaatttctttatcatgaggagatgtgatctgagcaccagtttcccagtaaaccttgtatccattgtcttccttgcggttgtgagaggcagtaatcatcacacctgcaactgctttgagcttctgaactgcatatggtacaaaaggtgtaggaacatatcttgaaaaaaggtacacaggaacatctttggccagcaagactgcagcagtgagtttagcaagcctctggctgctgcagctgctagttacttgaccccgagtgtcatacccaaccacaaagcctctctgcttgaagtctgagaaacatctctcaaggtatttgtacatcccctgtgttgactgtattactgtaaggtcattaatatagcaaaaccctgcccccatggcagaacgaagtcctgcagtcccaaaagtcattcggcaacaaagacgatctcgcagctccttgttcatcccattccgtaacaggttttcaatctgctcttttgttttgggattcttatcccagcggagccactgcccgatggccgtgtccagctgagggtccccggtgtggtagggggcgtggagcaggttggagttcagatccccctctgtgttttcagccatggcgaccagacaggcgtacgggccgggggccggcgaagacactgagttggggtggggggtggcttggggttcgctcaccagggtccaggcgtccccacctcactgaagggcatcggagaccaaccgcagggtgttcgtaacagctcctgccgcggcgtcagggaaccgggagagagggggtttatggccgcctgctccccagcggaccaggtccgggtctctgggcgaagtgactgaggcggtcgcgccgcgagagaacaacagtcccagat

SEQ ID NO: 13967 - RNA, 1683 nt, Homo sapiens
  source 1..1683: mol_type = other RNA
gctgggattacaggcatgagccaccgagcctggaccagaatcttacttctttcttgcaccatggtccttcgaggatcctgtcatgagtgaccttccatgtggtgattcagcggcccaggcgccttccatctcatggctctgccatcttctctggccttggggagtttcatctctagctcatccccaaagctcatgacgtagatgaaatattgtaactagctctgtagacagtttgcagtgtacatcttcccccaagcgatgccagcttctagttctggaggctgggaagtccaagatcacaagaccagcatctggcgagagccttcttgtgcaccatctcaaatgtaactgtggtggccagcatccaagatgaccatcagggattatcatctggcaatgatgcccgtgtctgatccctttccatgttggatggagctaagcgatctgtaggatattgcaaaagtggcaacatatagcttccaagcatagatcattaaagatgttgtgtctttctccttgctctctcttgagctgctctcttggggaagtcagccatcctgttgtgaggacgctgaagcaaccctgtgaattctttcttgtgatgatgtcaagaatctggggaccggctgtggctggggtctcgttggcatccagaaaccctcctgagccctcttgtgacaccaggatttgccgacagagcaaatgtgaggagaggcatcagaatttctctaagacttctgagctgagcaaccatctagaaggttggagctgctttatttggtggggaatgttagggaaaccagccccacaccacccagtgggtaccctgagtctggtggagacataggagttagaaagagacagaataagcatttaaaaggcgggttcaggggaccagaatatcggaggcttgctcacggcccagagctcttgagctctgccaaatttactggtttacaagctctttgttcttagggcagatgggagggggaggaagggatgaggaaaaggattaatcagtgaaggagaactcgtgagtcattccataagatgtgtagcagtggcggtttctgtgaatttccttgagcaaaggcgtgtgtctaaactacttaagatctttagcttatcaggactgaaatgggtgggagcgggtttaaggaggagccaagatgtttgattatactccactgcttcaagggagtgttgtctccctgagcaacctgtggaatgctgctgagtggttatgctcttggggcataaagacatgaaagcaataaggagacttttctccccagaggctgcccatggcttcccatgggtgtctcacacaggggagaccaactcaactggcaccccagaaacactttcccacatgttccccttttttgcctctattgatttttttttattaataactgccattgctattatggctcattcatggtgtctggtttctctcccaaggcaccatctgcatctgtagactaaaaacaagcaacataaacagacacaaaccaaaataaaatttgcaattgttgatccacctatggtttcaatccactttaaaggattggtattagaaaggccatcagaggctccagcaagaatatcagctccaggcaatagggtgagatgagcctgagatgcctcaaaaacttgttttttcagtttagcaatatctaa

SEQ ID NO: 13968 - RNA, 1545 nt, Homo sapiens
  source 1..1545: mol_type = other RNA
gctgggattacaggcatgagccaccgagcctggaccagaatcttacttctttcttgcaccatggtccttcgaggatcctgtcatgagtgaccttccatgtggtgattcagcggcccaggcgccttccatctcatggctctgccatcttctctggccttggggagtttcatctctagctcatccccaaagctcatgacgtagatgaaatattgtaactagctctgtagacagtttgcagtgtacatcttcccccaagcgatgccagcttctagttctggaggctgggaagtccaagatcacaagaccagcatctggcgagagccttcttgtgcaccatctcaaatgtaactgtggtggccagcatccaagatgaccatcagggattatcatctggcaatgatgcccgtgtctgatccctttccatgttggatggagctaagcgatctgtgaattctttcttgtgatgatgtcaagaatctggggaccggctgtggctggggtctcgttggcatccagaaaccctcctgagccctcttgtgacaccaggatttgccgacagagcaaatgtgaggagaggcatcagaatttctctaagacttctgagctgagcaaccatctagaaggttggagctgctttatttggtggggaatgttagggaaaccagccccacaccacccagtgggtaccctgagtctggtggagacataggagttagaaagagacagaataagcatttaaaaggcgggttcaggggaccagaatatcggaggcttgctcacggcccagagctcttgagctctgccaaatttactggtttacaagctctttgttcttagggcagatgggagggggaggaagggatgaggaaaaggattaatcagtgaaggagaactcgtgagtcattccataagatgtgtagcagtggcggtttctgtgaatttccttgagcaaaggcgtgtgtctaaactacttaagatctttagcttatcaggactgaaatgggtgggagcgggtttaaggaggagccaagatgtttgattatactccactgcttcaagggagtgttgtctccctgagcaacctgtggaatgctgctgagtggttatgctcttggggcataaagacatgaaagcaataaggagacttttctccccagaggctgcccatggcttcccatgggtgtctcacacaggggagaccaactcaactggcaccccagaaacactttcccacatgttccccttttttgcctctattgatttttttttattaataactgccattgctattatggctcattcatggtgtctggtttctctcccaaggcaccatctgcatctgtagactaaaaacaagcaacataaacagacacaaaccaaaataaaatttgcaattgttgatccacctatggtttcaatccactttaaaggattggtattagaaaggccatcagaggctccagcaagaatatcagctccaggcaatagggtgagatgagcctgagatgcctcaaaaacttgttttttcagtttagcaatatctaa

SEQ ID NO: 13969 - RNA, 10739 nt, Homo sapiens
  source 1..10739: mol_type = other RNA
gctgggattacaggcatgagccaccgagctcagccaaagatgtttttcttgattagttaataaattacatttagttttaagatatgcaactgaagcaaaagtataccaatacggaatcgggcaaaacgatttttgcccgatacacaaacgctgaggtaaatttgaaactaatttcttttctcattgtgcaacataagtactaatgtgtggtttgaaattatattccagtcttataaactggaaaggttaagcgtcaataatttattgtcgcctttgcaaatgcttagatatattttttagttgtaattgtgtcctgcttatttttctcacattcttccgtactggcctgggaactctcctgttctttgatcagagatgtagtacaacgtcgtttcagtctgagataatcttctgaactggtgggagcagtcctagtggattcactgacagatataaattgtttttctcctgttgaaccagacaaaagagcttgggtatttatcaatgcaagttcttcgtcagctattgaattactttccaaaagagaaatttcattgaattttttaaatggagtcatctgaggagaattcagttcttttttctttatgggtgtttcgtatttggtgccacaactccttggtggctgaaatgccttctgtgcagccggagaaacaaatgtacaaatgggactaacaggtggaggtaaaggcagtctactcaagaaatccaaggctcttctctttttgcagttcttttggtcatcaatctctttctcccctttacaagactttgaagtcatctgggctgagacaggtgtggaaacagacttccttttggccatacaaagtgataaaggactttgataatatatctcacaattaggagaagacatcagaagcttgtttcctgtaccaggaatgatttgagcagtgtacggccctgaagtacagtctttagttggggtggaccacttgggatcatttgcatgcagtatatgcataagcttgttttctgcttcattgcaaagtatgtcaatattctcaacagtatttttcattttgttgaatgtctcttgaaagtggccctcttttggactagcagaaaacacagaaaaatctccagcaaataaagtaagaaggcctgatttggattctggtcgccactggaggttgcttgcagcaattaacatatgaggcttaataatgtcctcattaaggtctatccaaaactttattgccagtaaattgtaacattcgtctgacaaatagacgaaaggggcaagtcctgtttttttcacaacagaaacgacaaatcctattaggtccacctcagaacaagatggctgaaagtctggatctaaaaatttgctgaagtgaaggggctcccgtggctggtaaatctgaaataaaatttcatctgaaaccggtagttgttgatactgagttttttttgtcgctgctaactgtatgttagctctttcagatttacttttagattttgaagttgcaagatgataaattctgtatctctttccttctgttaacagagaatataaatctgatgatggacgccaaatactcagtataactgaatctttttctttttttgaatagcttacaatacgcaacttccacacggttgtgacatcccttgataaaccttgttccttttgttcagcagattccatggccttcctaatttccaactggatctgagcttgtttcttatcattcaacatttgcctgtgattattcaaggctcttaactgctcttcactgaaataaccctcaaggtaagctgggtctgctgcattcttcactgcttcataaagctctgcaccatcttgcaaagcacgaacttgctgtcttgttagtgcacgtgatggtaaatatggttttgttgtgttttcttcatgttcttcaaattcctcctgaattttagtgaataaggcttctagtctcttttgttgggcctccacatattttgctgcttccttttcttcctctctttcattgcgaaatatgtataatccagatgatgtcttctccatccactgtatagggtatgctctttgaataattacatcaacacaaccaacatttcctccatcactgaaaagcgatgataagggcagaggaaaaggtctagggtcaggaaagaatccaagtttggtataccagcgagcaggccgagtactgttagcagaaatctttaacataagagattctggggcttcaagaggtgtacaggcatcaggagagcccaccagttctgctccatgaagaataatcttctgaccaactgtcagtctgccattctttaagacagctaagaggggaggatctaactgggccttaacagcataccacccatctgtaagttcaataatggccactttttgggtatctgcactactagttttattgctagaagtttcagatatatttgcgctcaatgaaattatgtcagaaacacagagaacaagtgtttttgcagctgtgtcatccctttccattatcttttttatagccgatcttctgcttctatcaatttccgtatcatatctgtattttagttgaagaagcaccctttctgggcttaggcatctattagcaaattccttaggaaaggcacattccatagctgccagtttccatatgatccatctatagtgattataaacccaaattctagaaataagctttggatccacacctggagtgtcacacagagccctataaaattcttcttttccagcctttccatcattggagggtatgagccatccaccatcagccaactgtattccttttccagtccataaactttccttaccaaaataatcttcagtgtgaaactgaaaagactctgcatttttgctgttaatttttatgcaatgtttagaaacgccatacgtatacagctgtttatgagaacacgcagagggaacttggcctcctactgctgctttcagagagattcgaggcagagtggatgtttttgcaagatacagactgcctggctgtggaaagacgcgttgcctttgtttcttcttaattcgcatatcctgtatatctctggcattctgaagacttgtaattaaatctaaaggttcttcttcacactttgtgaaagttacagctactgcttgattggagttgtttttgttaaactgatgaatctcattgtcattaatcttatttttactatcatcagagccatgtccatcaatgttttgcttttgtctgttttcctccaagttaatattcctaacacactgttcaactctgtgaaaatgtgatttagttttaaaaggtggaacaaagactttggttggtctgcctgtagtaatcaagtgtctcattttttcatttcttgtagcagaaacttgataaaatggatgtcctgaaactgctaaattgcttgaagatttttccaaagtcagatgttcatacaaatgagatttagacagaaattcttgaccaggtgcggtaaaatttggattctgtatctcttgacgttccttagttgtgcgaaagggtacacaggtaatcggctctaaagaaacatgatgcataaacaatcttcgatcttttattgtgccatctggagtgctttttgaagcctttaaggatttttcttgattttctattatcctgtcaaattcatttaataagtttcttttgattgagggttctcccactaagataaggggctctcctcttctttttccaattcttgaatttgacaaaaccatttcctcattttcgggacatgtaaaaagagaatgtgtggcatgacttggcagtttagaatctgtcagttcatcatcttccataaaagctttagcaatttctactgcttctgtttcaaagtagttttctgaatctttggagtaagtagaacaaacttctatatttgttttcacaggaacatcagaaaaagtttcagttttaccaatttccatttttacgtttttaggtgaagcctgttcttttcccaaaacatgaatgttctcaacaagtgacactttggttcctaataccaactgttgtttgtcttgttgaaattgagagagatatggagaaactttaatagagtgattattttctgaagaaccaccttcaacatttaagttatttgataatttaaattctttactgcaggttttttccatttctgagtttacacagtgctctgggtttctcttatcaacacgaggaagtatttttgatacattttgtctagacgtaggtgaatagtgaagactatgctcagttctgattaaatcaaattcctctaacactcccttaactttgtgtaaggaactttctaaaatggaaacttgctttccacttgctgtactaaatccagagaaagcagatgaatttaccacattatatgaaaagcctttttgggatattaaatgttctggagtacgtatagcagtattttcttctcttgtgagctggtctgaatgttcgttacttttaaacaatactttggaaaagacttgcttggtactatcttctatttcagaaaacacttgtcttgcgttttgtaatgaagcatctgatacctggacagattttccacttgctgtgctaaaaatcccacaagtatttgcagatgagactgacttatgaagcttccctatactacatttacatatatctgaagtttccaaactaacatcacaaggtgatattttagaaactttctccaatccagacatattttggttatgttgtaaaatttcttcactctgaatgtcagcaaaaaccttatgtgaatgcgtgctacattcatcattatctagagagttatgaagaatatcctctgaatcatccaatgcctcgtaacaacctgccataattttcgtttggcaaatttttgatttattctcgttgttttccttaattactttactgaaactgtctgtaaatatgtctttcacttttttaattgtttcatgtgaaacacaaacgattttaccactggctatcctaaatgcaggtggccctacctcaaaattattactattagatatggacaatttaatggctgcatttttatttttgcagggtgaagagctagtcacaagttcctcaacgcaaatatcttcatttacagtttgtgggtatgcatttgcatcttttacattggatattactttggaaaaactagtgtttttttgatcttcaacattcttcaatactggctcaataccagaatcaagtttattttttgagagatatcctgaatcattatatacctcatcagaatggtaggaatagctgttagacatgctactgttacttaaataagtatcttgtttttcggagagatgatttttgtcattttcagctatagtactgtttgaattattttcatacaaataatttcctacataatctgcagtatttattctttctggttgaccatcaaatattccttctctaagccatttttttgcttcaagtaatgaagtctgactcacagaagtttttctactacaacttgtgtaaaaagctaaggctgaattttcaatgactgaataaggggactgatttgtgtaacaagttgcaggactttttgctgtttctttttctacattttcatgtactttaactttcaaaaagatactttttgatgttttgagattttcagtttgtctacataaattatcacttaagagcttaggtggcaccacagtctcaatagaaacaaggtttttatcattattgagagaattctgcatttctttacactttggggcagctgtgatctcaatggtctcacatgctaattcaaggtctttacaggcctctctgtactttagggtctttgcccattgatggctaaaactggtgatttcactagtaccttgctctttttcatcaaaaaggtttttcactttgtccaaagattcctttgcaattttaacttttttcccgctagctgtatgaaaacccaatagagtaggttctttgatcttttcatcacgttcgggttgtccctggaaggtcactagttgatttccagtaccaactgggacactttctttcagtattttgtgtttaactatgtctgtttcctcataacttagaatgtccattttgttctttcttatgtcagaatgtaattcagaatttaaggaaaagttatgcaattcttctggtttctgatcaaagaaatttacaattttattaaatgactctttggcgacactaatatttttcccacttgcagtctgaaaaaatgtatcagaagtctcaaaatcttttatattttgctccgttttagtagcagttaactgttctttatttgaagtattaccatgacatgcttcttgagctttcgcaacttccaaaaaagttaaatctgacaaatcttctttaatctgagtgtttccctccttcataaactggccagataatttaagacatatgttgtgctgatcagtaaatagcaagtccgtttcatctttatgaatacaaacagtatcatttttacttgaatcactgccatcaaattctaagttatgagaatttctactggcagcagtatatttgttatcttcattttcagtatttctcttgtaattttcagtaatttcttcaacaaaagtgccagtagtcatttcaatattattttgtaatatcagttggcatttattatttttttcacttacagttttatcattatgattttctatcttaaacattgaaacaacagaatcatgacatttacttgaagataaacttattggatgtacctctgcagaagtttcctcactaatattctcaatatcactaaacagtttcacagctttttgcagagcttcagtagaaacattcagttttgtgccatgagcagaataaaagcccctaaaccccacttcattttcatctgttaaataaccagaagcacttttgttacagtcatttttcaacaggccagcaaacttccgtttaatttcaactgtaccttcaaattgcttgctgctgtctacctgaccaatcgatggggcattcattatgacatgaagatcagcatctctgcattcctcagaagtggtctttaagatagtcatctggttttcaggcacttcaaatgtactcttctgcaatatgtagcttggttttctaaactgagtaaattcaaactgacttcctgattcttctaatatagtagaaagttctgtaatttctgccttttggctaggtgttaaattatggtttgaattaaaatcctgcttggaaaataacatctgaggggttatatgactatttttacaatcagaaacaactacactactctgtaaatgtgcagatacagtattaattgactgaggcttgctcagtttcttttgattatctaatgccaaggtatttacaatttcaacacaagctaaactagtaggatattgttcttcaatatctttgaagaacattttgctcttcttaatgttatgttcagagagcttgatttccttatttgaagctgttctgaagctacctccaaaactgtgatttgaaattggacctaagagtcctgcccatttgttcatgtaatcattatttttttctggtattttatctatattcaaggagatgtccgattttaaatcttgacctagagtcatttttatatgctgctttacactatttttgttctcctctgcaagaacataaaccaaatcttttttaattgacacttgggttgcttgtttatcacctgtgtctccatataaaaccatggtagagttcttgaaaatgggttcgtttacacaagtcaagtctgtttcatgaagttccttagtatttcctaaagcaagattattcctttcattagctacttggaagacaaaattattctcattgtctgagaaaagttcttcagagtctggattgacagttatttttgaaattgaagtagtttcttcttgatttttttggattactcttagatttgtgttttggttgaattgtacctttcttgaaggtgatgctactctcatgtatttttcaggtggcaacagctcaacgtttttataattttcatttaaagcacatacatcttgattcttttccatgggaatatttttggttaattcaacatcagattcataattgttacctttgagcttgtctgacattttgtatgattctttgcctctagaaatcatgactaggtttgacagaacatccttggaagtaggagttaaaataagagtgctggcattttcatgatcatataaaagacttttctgggattgaaagtcagtatcactgtattccacttttgaatgttgtactgggtgacatgctgcagccaagacctcttcttttatatctgaaacttttttgctttttggatcattttcacactgtccttcctgcaggcatgacagagaatcagcttctggggtaataaataactgtagtttttccttattacattttgcttctttataatcaagatcctgagagattactgtattattagaacatgtttcatttctagaacatttcctcagaattgtcccaaaagagctagttaaggacaaagttggttcttcagaatcattctgtgaacagcttcttttcacagaagaatgcaataaacctgaatcagcatttgcaaatgtaagtggtgcttcaaaagcatttgcttcaaactgggctgaacagttaattagttctgatttttggtctttcggtattttttttcctttataagatgtttcatcatgtatagcataaataaacttatttgttttctttttcaaagtggatattaaacctgcattcttcaaagctacagaattctgtgtggtggtggctggccagcttccattatcaattaaatttggacataaggagtcctccttctgtgagcaaacagtatgtatttccagtccactttcagaggcttcagtttcttttttaaagtttggatcagtcatatgacctgaaaaacttgcattgaaagtctctttaggtgattctcttattctgaatatagactttttgataccctgaaatgaagaagccactggagaagttccagatattgcctgctttactgcaagaatgcagtctgtatgagattcaagatgctgctcttcatctctcttatttaccactgtttcctcatttaatggcttctctgattttggtaggctagaaatacgtggcaaagaattctctgaagtaagaaaatctttctttcttttgttctctgtgtctaataggtctttttctgaaatattttggtcacatgaagaaatatgcaataggggtattttctccatctgggctccatttagacctgaaagggttagttgagaccattcacaggccaaagacggtacaacttccttggagattttgtcacttccactctcaaagggcttctgatttgctacatttgaatctaatggatcagtatcatttggttccacttcagatacaaatgagtatttttctttcacttggtttttagatttttcacattcatcagcgtttgcttcatggaaaatttttttcctagtcttgctagttcttactttttgtagattttttgttctacatttagaaaaacataatgaaaaactatcttcttcagaggtatctacaactgtttcatatacttcatcttctaggacatttggcattgactttccaatgtggtctttgcagctatttactttaaatgaattccctgatgtttttccaaatccatgacttgcagcttctctttgatttgtgttttcactgtctgtcacagaagcgataaatctatcatttttcttcagactttcatcatgattggaaaaatagcttttcacattagcagtagtatcatgaggaaatacagtttcagatgcttcttcatttctgactatgagcacagtagaactaagggtgggtggtgtagctaaagaacttgaccaagacatatcaggatccacctcagctcctagactttcagaaatatgttttggtgtctgacgacccttcacaaactttggtgtatgaaacaaactcccacataccactgacttatctctttgtggtgttacatgtgtacattgtagaacaacaggactttcactaagacaagaatttagaagtggacaggaaacatcatctgcttgatccattttagttttcactgtgcgaagacttttatgtctactattgggaacattccttcctaagtctaatttgaatttatctaattcttttacaggagattggtacagcggcagagtcagcccttgctctttgaatattattggagttgaagccagctgattataagatggtttcctttgtggagttttaaataggtttggttcgtaattgttgtttttatgttcagattcttctgcaggttcagaattatagggtggagcttctgaagaaagttcttcaaaccaattaagacttattggtcctaaatctgctttgttgcagcgtgtcttaaaaatttcaaaaaatgttggcctctctttggatccaataggcatttttacctacgatattcctccaatgcttggtaaataagtccgctccagaggtgcagttcttttttggccggagtaagctgacaaaaaccgcgccggtcacaaatctgtcccctcacgcttctcccggcggcgacccaccgccgcaaaagacacccgaggcgcagcagaggcgcagcagtgccacagcggctccgcctct

SEQ ID NO: 13970 - RNA, 1129 nt, Homo sapiens
  source 1..1129: mol_type = other RNA
gctgggattacaggcatgagccaccgagctcagccctaattagttattttctgagtatgccactaacaaatgaaatgattaaataagtcacattttctaggcccattttttgacctttatacaacactgtcacttgatttttgtaacatcagaataggaacaatgatgcatctccacaggctgcaaagacagtgagtagacaggaagggagcaggcttatggaggagcacagggacaagttccccatctaggcgatgccttccccagactgtgtcctcacagtcctcacagtgggcagtgacgtgtcctctcctgtgctgcctgccccttgctcatgctggcagcctaattcttcctgaaagcccatccactggacagtctgccatggtttctgcatgtgctgacatcaccaagtgttatttaactggcttagaaacttcaatcatactgcctgaccctggagctcagaagaaacatcaagaatcctggaaacacacgggccaagtttcctgtgaaggcacatcagttctcaatgataaggtctacaaacatcggggactcttcacatatatgtttaatgctgctgtcattcaacttttataagcttcagattccatgttttgttgttgtggaatagaagctcccaaaaatggtcatcttcattttcctggctgctctctaacacgtcatcaactttccatttcctttctgggtggcactggcttgggaatcctttttctaatatccagggctcttctccttgctcgatcttaaagatcacttctggtttagtaatgcaataccctactgagacaagattgctataattttccaggatcacatctctgtatagaatcttctgagcagggtccagcagataccactcttcctgagtgaagtccacacatacatccttgaatgacacttgttcccgccgctcctcgccgcctccggaggcgagggattgtttcccacaagggactggagtccagggaaggactcgcctggagcgggaggcggggatgcacatgcgcagagggagaggccgagcgcccgagttaggctggtggatgcgatgcggggcttggaagcggcgctagacggtgcctgtcagctctggccgcaaccc

SEQ ID NO: 13971 - RNA, 1497 nt, Homo sapiens
  source 1..1497: mol_type = other RNA
gctgggattacaggcatgagccaccgagctcagccctaattagttattttctgagtatgccactaacaaatgaaatgattaaataagtcacattttctaggcccattttttgacctttatacaacactgtcacttgatttttgtaacatcagaataggaacaatgatgcatctccacaggctgcaaagacagtgagtagacaggaagggagcaggcttatggaggagcacagggacaagttccccatctaggcgatgccttccccagactgtgtcctcacagtcctcacagtgggcagtgacgtgtcctctcctgtgctgcctgccccttgctcatgctggcagcctaattcttcctgaaagcccatccactggacagtctgccatggtttctgcatgtgctgacatcaccaagtgttatttaactggcttagaaacttcaatcatactgcctgaccctggagctcagaagaaacatcaagaatcctggaaacacacgggccaagtttcctgtgaaggcacatcagttctcaatgataaggtctacaaacatcggggactcttcacatatatgtttaatgctgctgtcattcaacttttataagcttcagattccatgttttgttgttgtggaatagaagctcccaaaaatggtcatcttcattttcctggctgctctctaacacgtcatcaactttccatttcctttctgggtggcactggcttgggaatcctttttctaatatccagggctcttctccttgctcgatcttaaagatcacttctggtttagtaatgcaataccctactgagacaagattgctataattttccaggatcacatctctgtatagaatcttctgagcagggtccagcagataccactcttcctgagtgaagtccacacatacatccttgaatgacacttgttcctgggatttgttcattttccgctcttagtggaggaaggagaggtgtccatgtgtggctccgatatatgctgagctcagacatgacacttttcactgagtgaatgtaaatatttcttattgatttattaccaatttaggttctctctcttcttaaatttgtcccagaccttgcaccagcacacagactccgacggcttcaggatactgtgccatgattacacataatacataagcgaacgcgaaacgtgtaaataattacttgggataggagggcggtcagagccagcaggggccctggtggtcagctaggccagccccttcgctcctgcactccacgggcagagaggcccttggggccggtgcaggagccgtctccctcgggctctcccagggaacgcacacccaataaatacagcacctaaacaatgaaagtgctcaaaacaaccccaggcggcaagtattcctaatatccgtaatttacagagaggaaaaccgagtctcccgtggataattgtgtctaattcatttgtcgcggacctggcgcagtcgctctcccccgcagcccc

SEQ ID NO: 13972 - RNA, 1309 nt, Homo sapiens
  source 1..1309: mol_type = other RNA
gctgggattacaggcatgagccaccgagctcagccctaattagttattttctgagtatgccactaacaaatgaaatgattaaataagtcacattttctaggcccattttttgacctttatacaacactgtcacttgatttttgtaacatcagaataggaacaatgatgcatctccacaggctgcaaagacagtgagtagacaggaagggagcaggcttatggaggagcacagggacaagttccccatctaggcgatgccttccccagactgtgtcctcacagtcctcacagtgggcagtgacgtgtcctctcctgtgctgcctgccccttgctcatgctggcagcctaattcttcctgaaagcccatccactggacagtctgccatggtttctgcatgtgctgacatcaccaagtgttatttaactgtacaggagtgccaagaatgtcttcagtgaacaggcagttccagacatgctctttcctggccttttccactctgctctgaggctctgctgaaaggtctcagatcagaagtgtgaccttccacgtgggttcttagggactactccttattacctcaaaagctactttattccaaggatgctggcttagaaacttcaatcatactgcctgaccctggagctcagaagaaacatcaagaatcctggaaacacacgggccaagtttcctgtgaaggcacatcagttctcaatgataaggtctacaaacatcggggactcttcacatatatgtttaatgctgctgtcattcaacttttataagcttcagattccatgttttgttgttgtggaatagaagctcccaaaaatggtcatcttcattttcctggctgctctctaacacgtcatcaactttccatttcctttctgggtggcactggcttgggaatcctttttctaatatccagggctcttctccttgctcgatcttaaagatcacttctggtttagtaatgcaataccctactgagacaagattgctataattttccaggatcacatctctgtatagaatcttctgagcagggtccagcagataccactcttcctgagtgaagtccacacatacatccttgaatgacacttgttcccgccgctcctcgccgcctccggaggcgagggattgtttcccacaagggactggagtccagggaaggactcgcctggagcgggaggcggggatgcacatgcgcagagggagaggccgagcgcccgagttaggctggtggatgcgatgcggggcttggaagcggcgctagacggtgcctgtcagctctggccgcaaccc

SEQ ID NO: 13973 - RNA, 1498 nt, Homo sapiens
  source 1..1498: mol_type = other RNA
gctgggattacaggcatgagccaccgagctcagccctaattagttattttctgagtatgccactaacaaatgaaatgattaaataagtcacattttctaggcccattttttgacctttatacaacactgtcacttgatttttgtaacatcagaataggaacaatgatgcatctccacaggctgcaaagacagtgagtagacaggaagggagcaggcttatggaggagcacagggacaagttccccatctaggcgatgccttccccagactgtgtcctcacagtcctcacagtgggcagtgacgtgtcctctcctgtgctgcctgccccttgctcatgctggcagcctaattcttcctgaaagcccatccactggacagtctgccatggtttctgcatgtgctgacatcaccaagtgttatttaactgtacaggagtgccaagaatgtcttcagtgaacaggcagttccagacatgctctttcctggccttttccactctgctctgaggctctgctgaaaggtctcagatcagaagtgtgaccttccacgtgggttcttagggactactccttattacctcaaaagctactttattccaaggatgctggcttagaaacttcaatcatactgcctgaccctggagctcagaagaaacatcaagaatcctggaaacacacgggccaagtttcctgtgaaggcacatcagttctcaatgtgttttgttgttgtggaatagaagctcccaaaaatggtcatcttcattttcctggctgctctctaacacgtcatcaactttccatttcctttctgggtggcactggcttgggaatcctttttctaatatccagggctcttctccttgctcgatcttaaagatcacttctggtttagtaatgcaataccctactgagacaagattgctataattttccaggatcacatctctgtatagaatcttctgagcagggtccagcagataccactcttcctgagtgaagtccacacatacatccttgaatgacacttgttcctgggatttgttcattttccgctcttagtggaggaaggagagctctctcttcttaaatttgtcccagaccttgcaccagcacacagactccgacggcttcaggatactgtgccatgattacacataatacataagcgaacgcgaaacgtgtaaataattacttgggataggagggcggtcagagccagcaggggccctggtggtcagctaggccagccccttcgctcctgcactccacgggcagagaggcccttggggccggtgcaggagccgtctccctcgggctctcccagggaacgcacacccaataaatacagcacctaaacaatgaaagtgctcaaaacaaccccaggcggcaagtattcctaatatccgtaatttacagagaggaaaaccgagtctcccgtggataattgtgtctaattcatttgtcgcggacctggcgcagtcgctctcccccgcagcccc

SEQ ID NO: 13974 - RNA, 1449 nt, Homo sapiens
  source 1..1449: mol_type = other RNA
gctgggattacaggcatgagccaccgagctcagccctaattagttattttctgagtatgccactaacaaatgaaatgattaaataagtcacattttctaggcccattttttgacctttatacaacactgtcacttgatttttgtaacatcagaataggaacaatgatgcatctccacaggctgcaaagacagtgagtagacaggaagggagcaggcttatggaggagcacagggacaagttccccatctaggcgatgccttccccagactgtgtcctcacagtcctcacagtgggcagtgacgtgtcctctcctgtgctgcctgccccttgctcatgctggcagcctaattcttcctgaaagcccatccactggacagtctgccatggtttctgcatgtgctgacatcaccaagtgttatttaactgtacaggagtgccaagaatgtcttcagtgaacaggcagttccagacatgctctttcctggccttttccactctgctctgaggctctgctgaaaggtctcagatcagaagtgtgaccttccacgtgggttcttagggactactccttattacctcaaaagctactttattccaaggatgctgggacaaggggacaaagtaaatttagttggaaccttcaatctgaccttcagataacacactttccctgagaatcaaggcctgggccatccatgaattcaaacaaagtcccccaaggacaaatgctggacaaggcttacctggcttagaaacttcaatcatactgcctgaccctggagctcagaagaaacatcaagaatcctggaaacacacgggccaagtttcctgtgaaggcacatcagttctcaatgataaggtctacaaacatcggggactcttcacatatatgtttaatgctgctgtcattcaacttttataagcttcagattccatgttttgttgttgtggaatagaagctcccaaaaatggtcatcttcattttcctggctgctctctaacacgtcatcaactttccatttcctttctgggtggcactggcttgggaatcctttttctaatatccagggctcttctccttgctcgatcttaaagatcacttctggtttagtaatgcaataccctactgagacaagattgctataattttccaggatcacatctctgtatagaatcttctgagcagggtccagcagataccactcttcctgagtgaagtccacacatacatccttgaatgacacttgttcccgccgctcctcgccgcctccggaggcgagggattgtttcccacaagggactggagtccagggaaggactcgcctggagcgggaggcggggatgcacatgcgcagagggagaggccgagcgcccgagttaggctggtggatgcgatgcggggcttggaagcggcgctagacggtgcctgtcagctctggccgcaaccc

SEQ ID NO: 13975 - RNA, 1392 nt, Homo sapiens
  source 1..1392: mol_type = other RNA
gctgggattacaggcatgagccaccgagctcagccctaattagttattttctgagtatgccactaacaaatgaaatgattaaataagtcacattttctaggcccattttttgacctttatacaacactgtcacttgatttttgtaacatcagaataggaacaatgatgcatctccacaggctgcaaagacagtgagtagacaggaagggagcaggcttatggaggagcacagggacaagttccccatctaggcgatgccttccccagactgtgtcctcacagtcctcacagtgggcagtgacgtgtcctctcctgtgctgcctgccccttgctcatgctggcagcctaattcttcctgaaagcccatccactggacagtctgccatggtttctgcatgtgctgacatcaccaagtgttatttaactgtacaggagtgccaagaatgtcttcagtgaacaggcagttccagacatgctctttcctggccttttccactctgctctgaggctctgctgaaaggtctcagatcagaagtgtgaccttccacgtgggttcttagggactactccttattacctcaaaagctactttattccaaggatgctgggacaaggggacaaagtaaatttagttggaaccttcaatctgaccttcagataacacactttccctgagaatcaaggcctgggccatccatgaattcaaacaaagtcccccaaggacaaatgctggacaaggcttacctggcttagaaacttcaatcatactgcctgaccctggagctcagaagaaacatcaagaatcctggaaacacacgggccaagtttcctgtgaaggcacatcagttctcaatgataaggtctacaaacatcggggactcttcacatatatgtttaatgctgctgtcattcaacttttataagcttcagattccatgttttgttgttgtggaatagaagctcccaaaaatggtcatcttcattttcctggctgctctctaacacgtcatcaactttccatttcctttctgggtggcactggcttgggaatcctttttctaatatccagggctcttctccttgctcgatcttaaagatcacttctggtttagtaatgcaataccctactgagacaagattgctataattttccaggatcacatctctgtatagaatcttctgagcagggtccagcagataccactcttcctgagtgaagtccacacatacatccttgaatgacacttgttcctgggatttgttcattttccgctcttagtggaggaaggagagccgccgctcctcgccgcctccggaggcgagggattgtttcccacaagggactggagtccagggaaggactcgcctggagcgggaggcggggatgcacat

SEQ ID NO: 13976 - RNA, 1368 nt, Homo sapiens
  source 1..1368: mol_type = other RNA
gctgggattacaggcatgagccaccgagctcagccctaattagttattttctgagtatgccactaacaaatgaaatgattaaataagtcacattttctaggcccattttttgacctttatacaacactgtcacttgatttttgtaacatcagaataggaacaatgatgcatctccacaggctgcaaagacagtgagtagacaggaagggagcaggcttatggaggagcacagggacaagttccccatctaggcgatgccttccccagactgtgtcctcacagtcctcacagtgggcagtgacgtgtcctctcctgtgctgcctgccccttgctcatgctggcagcctaattcttcctgaaagcccatccactggacagtctgccatggtttctgcatgtgctgacatcaccaagtgttatttaactgtacaggagtgccaagaatgtcttcagtgaacaggcagttccagacatgctctttcctggccttttccactctgctctgaggctctgctgaaaggtctcagatcagaagtgtgaccttccacgtgggttcttagggactactccttattacctcaaaagctactttattccaaggatgctgggacaaggggacaaagtaaatttagttggaaccttcaatctgaccttcagataacacactttccctgagaatcaaggcctgggccatccatgaattcaaacaaagtcccccaaggacaaatgctggacaaggcttacctggcttagaaacttcaatcatactgcctgaccctggagctcagaagaaacatcaagaatcctggaaacacacgggccaagtttcctgtgaaggcacatcagttctcaatgtgttttgttgttgtggaatagaagctcccaaaaatggtcatcttcattttcctggctgctctctaacacgtcatcaactttccatttcctttctgggtggcactggcttgggaatcctttttctaatatccagggctcttctccttgctcgatcttaaagatcacttctggtttagtaatgcaataccctactgagacaagattgctataattttccaggatcacatctctgtatagaatcttctgagcagggtccagcagataccactcttcctgagtgaagtccacacatacatccttgaatgacacttgttcccgccgctcctcgccgcctccggaggcgagggattgtttcccacaagggactggagtccagggaaggactcgcctggagcgggaggcggggatgcacatgcgcagagggagaggccgagcgcccgagttaggctggtggatgcgatgcggggcttggaagcggcgctagacggtgcctgtcagctctggccgcaaccc

SEQ ID NO: 13977 - RNA, 1859 nt, Homo sapiens
  source 1..1859: mol_type = other RNA
gctgggattacaggcatgagccaccgagctcagccctaattagttattttctgagtatgccactaacaaatgaaatgattaaataagtcacattttctaggcccattttttgacctttatacaacactgtcacttgatttttgtaacatcagaataggaacaatgatgcatctccacaggctgcaaagacagtgagtagacaggaagggagcaggcttatggaggagcacagggacaagttccccatctaggcgatgccttccccagactgtgtcctcacagtcctcacagtgggcagtgacgtgtcctctcctgtgctgcctgccccttgctcatgctggcagcctaattcttcctgaaagcccatccactggacagtctgccatggtttctgcatgtgctgacatcaccaagtgttatttaactgtacaggagtgccaagaatgtcttcagtgaacaggcagttccagacatgctctttcctggccttttccactctgctctgaggctctgctgaaaggtctcagatcagaagtgtgaccttccacgtgggttcttagggactactccttattacctcaaaagctactttattccaaggatgctgggacaaggggacaaagtaaatttagttggaaccttcaatctgaccttcagataacacactttccctgagaatcaaggcctgggccatccatgaattcaaacaaagtcccccaaggacaaatgctggacaaggcttacctggcttagaaacttcaatcatactgcctgaccctggagctcagaagaaacatcaagaatcctggaaacacacgggccaagtttcctgtgaaggcacatcagttctcaatgtgttttgttgttgtggaatagaagctcccaaaaatggtcatcttcattttcctggctgctctctaacacgtcatcaactttccatttcctttctgggtggcactggcttgggaatcctttttctaatatccagggctcttctccttgctcgatcttaaagatcacttctggtttagtaatgcaataccctactgagacaagattgctataattttccaggatcacatctctgtatagaatcttctgagcagggtccagcagataccactcttcctgagtgaagtccacacatacatccttgaatgacacttgttcctgggatttgttcattttccgctcttagtggaggaaggagagctgaaggattagaaaggaagaatgtcaggagagccttcgccggccttgcagttcggagattcacctgcctatacaggtccacacacaagatacttacgtgtccatgtgtggctccgatatatgctgagctcagacatgacacttttcactgagtgaatgtaaatatttcttattgatttattaccaatttaggttctctctcttcttaaatttgtcccagaccttgcaccagcacacagactccgacggcttcaggatactgtgccatgattacacataatacataagcgaacgcgaaacgtgtaaataattacttgggataggagggcggtcagagccagcaggggccctggtggtcagctaggccagccccttcgctcctgcactccacgggcagagaggcccttggggccggtgcaggagccgtctccctcgggctctcccagggaacgcacacccaataaatacagcacctaaacaatgaaagtgctcaaaacaaccccaggcggcaagtattcctaatatccgtaatttacagagaggaaaaccgagtctcccgtggataattgtgtctaattcatttgtcgcggacctggcgcagtcgctctcccccgcagccccgcctcctccccgcgggctcagggcac

SEQ ID NO: 13978 - RNA, 1215 nt, Homo sapiens
  source 1..1215: mol_type = other RNA
gctgggattacaggcatgagccaccgagctcagccctaattagttattttctgagtatgccactaacaaatgaaatgattaaataagtcacattttctaggcccattttttgacctttatacaacactgtcacttgatttttgtaacatcagaataggaacaatgatgcatctccacaggctgcaaagacagtgagtagacaggaagggagcaggcttatggaggagcacagggacaagttccccatctaggcgatgccttccccagactgtgtcctcacagtcctcacagtgggcagtgacgtgtcctctcctgtgctgcctgccccttgctcatgctggcagcctaattcttcctgaaagcccatccactggacagtctgccatggtttctgcatgtgctgacatcaccaagtgttatttaactgtacaggagtgccaagaatgtcttcagtgaacaggcagttccagacatgctctttcctggccttttccactctgctctgaggctctggcttagaaacttcaatcatactgcctgaccctggagctcagaagaaacatcaagaatcctggaaacacacgggccaagtttcctgtgaaggcacatcagttctcaatgataaggtctacaaacatcggggactcttcacatatatgtttaatgctgctgtcattcaacttttataagcttcagattccatgttttgttgttgtggaatagaagctcccaaaaatggtcatcttcattttcctggctgctctctaacacgtcatcaactttccatttcctttctgggtggcactggcttgggaatcctttttctaatatccagggctcttctccttgctcgatcttaaagatcacttctggtttagtaatgcaataccctactgagacaagattgctataattttccaggatcacatctctgtatagaatcttctgagcagggtccagcagataccactcttcctgagtgaagtccacacatacatccttgaatgacacttgttcccgccgctcctcgccgcctccggaggcgagggattgtttcccacaagggactggagtccagggaaggactcgcctggagcgggaggcggggatgcacatgcgcagagggagaggccgagcgcccgagttaggctggtggatgcgatgcggggcttggaagcggcgctagacggtgcctgtcagctctggccgcaaccc

SEQ ID NO: 13979 - RNA, 2182 nt, Homo sapiens
  source 1..2182: mol_type = other RNA
gctgggattacaggcatgagccaccgcaaccggcccccaggaattctttaatggttccagagagttctctggctaaagactgctgctgcatctgttaggcaatgttgacaatctcatcagaagtggtgctaccactgtgtttcatgtttttgtgtttctttctttctgtcggtggttcctgagggttgtgacgatcagggcagaggcagaaggcaccacctcaatctgggcctgtctgctgtggctggtcagtttcactatcatcctcagactcttccagtcaatggttggtgatgtcatcagcaaccatttttggagacagacccagggagctgaccttgggggccagtgcagatgtggcactgacttcaccactggtacacctcagatatacaactttgatctcgctggggtcaaacgtaggtggctgcggttggttgaactcaggttcaggatgactgaagcaagttgcacttggctttctctgagccgaaaaacgaaaggtgctcaggctcccagcaactcatgcactttattgcctcctcttggaaacatccttatgtcattgcgctatggccagagccctgaaggacatctgctctccttgggagctgctgagccagggtgcccgtgatgtcttcagaatccttcagtcccgactgcaggagaaacttggcacaggccaagtgctgacctgcacaggccagatgcagggctgatcgatttttttcatctttagaattgatgtcagctcccaaggataagagagtctgaattgtacttgtatgtccttccttagctgcataatgaagtgctgtgaggtgggttgatgtggctctcacatctacatcgacgccaagttcagagaccaagaatcggatggcttcgtcctgccctgtgacagctgccctgtgcagagcctgggcacccaggctgtcttctgctgaaaggcaagccccatgttcatcgaggagcagcctagcgacgtcgatgtgcccacactggattgcgtccatcaaggcggtgacgccacagttgtctctgtagtctggttcatattggcacctcttaagaagcaccttgactgcctccaaatggccatgcattgctgcagtatgcagaggagtccttctaattttgctctctgtcttccaggcacctgggcaaacagtgagcaggtactggaggatcagagggtcgccttctcgactggcaatgtggaaactgttccagccatctttgttcttcaggagtggattggcgccatgttccaccagctcctggatcacccccaggttcttccttgtgcaggccatcatcagaggagtccagtcggccttcttcaggcagtcgaccgctgccccccggcccagcaggtagcgcacgcagtctcggtggcccatggaggccgcctcgtgcagaggccgcttgtagtctcggttggtggcctcgatgtccatgccccaggcctcggccagataggccagcacgtcccgatgcccgtggcgcgcggcgcagtgcaggagggtatccccggccggccccgggcagcccccggccgcctgcagctcctccttcagggcgcgcagccggccctcctgcaccagcctgcagaggcgccgcgggtccccgggctgggccatcgccgcgggtcgggccgggctgcgcggggaggcggcgggcgggacaccggcggccgggcagggagaagccgagggcgagtgggactttccgcctcttcacgcaacctgccccgcgcgccccgaacccggcagaaccgcccctcacgcccccggctttgtccccggcagagccgcctcctcaaacccccggcctagtccgcaggcgggctgccccctcacagccccggcctgccccgcgtgggagaagccgcggttccgggcacggggcggtttttcctcagggacggagcggtccgggatgagcacggaggggcctggggatccgagagcgctggcgtccgccgtcctggagctgcagcggcccgtacgtgattcgggactgaacacgtaagggagtggggcgcgccgctacaccgcaaagccccaaagtggagggtccgggagggcgcgcacagcctcgcccggcgccgtgcagggtggctcctgaggcagccaggcccaagcgtgacctgccccgcacgcgtcctcagggccgcccc

SEQ ID NO: 13980 - RNA, 496 nt, Homo sapiens
  source 1..496: mol_type = other RNA
gctgggattacaggcatgagccaccgcaaccggcctaaacaggccttgcccaggcaatgagcatccagttagacaggttcttcaaggcctagtaatagttctctggttacaacggtgctcagcttgtctgctaggaatgggactcccatctggacatgtctaggtcagtgttccaaaatatggccagtatggaaggaggtcttatcacatgcttctggatggatggtctggaaggcccttggtgggctctgtgttggctagttggcttctggtggtccaggaggtcccaggcgatgggctctctagtaagccctctagggactccatcactctaacgaagatggagagtagggtcagtaccacacctaacaggtagaggttcaacacatgcttcatggctgaaaggaccctactcctctgcagagaaacagagctgccttctccttctgaaaggcctctggacccggagacaaaagcgccgtcagccgcagagcgc

SEQ ID NO: 13981 - RNA, 610 nt, Homo sapiens
  source 1..610: mol_type = other RNA
gctgggattacaggcatgagccaccgcaaccggcctaaacaggccttgcccaggcaatgagcatccagttagacaggttcttcaaggcctagtaatagttctctggttacaacggtgctcagcttgtctgctaggaatgggactcccatctggacatgtctaggtcagtgttccaaaatatggccagtatggaaggaggtcttatcacatgcttctggatggatggtctggaaggcccttggtgggctctgtgttggctagttggcttctggtggtccaggaggtcccaggcgatgggctctctagtaagccctctagggactccatcactctaacgaagatggagagtagggtcagtaccacacctaacaggtagaggttcaacacatgcttcatggctgaaaggaccctactcctctgcagagaaacagagctgccttctccttctgaaaggcctctggaccctccgggggaacagccgggagtggatcgccggctgtaggagcaggtcgtgcaggagtccggaggaaagtcggttactaagcaccagcgcagaagcttcccgccacaaaactcaccggagacaaaagcgccgtcagccgcagagcgc

SEQ ID NO: 13982 - RNA, 979 nt, Homo sapiens
  source 1..979: mol_type = other RNA
gctgggattacaggcatgagccaccgcacacagcctgcaaactttgctcctggtccatgggtaaaaggagctctcagccttgcagaaaccttctgttggtgccacctgtaggaatcagggtttcatccacaggcaaataagtatccgcttctatggtgacttcatggtcatttatatttggggaagcctggcctgccaggttgaagtaagaatggttggtcaggttgactggtgtggcctgactggcttgtgctctgtagttgactatgagctctccgccatccagggtgtatgtcacccagacttttaactctccggggtagccttcttcaccatctggactgatgcgcgagaactggacgccatttgacagcacccgaggggtccagagcactttatcaaaccctctgactcctccatgcagactgttgggttccttgttaatggccaggtgatactccttcccatccaccttgaaggttcctttggcgattcggttggccaccctcccaataactgctccaaagtatggctgcttttggaggtatccttccaactcggcgaagccaagcaccacgtccgaggctctcccctgcctgtctttgacctctagggctgtgatcgtgcagccccaggagatgatgtccactctcaagaggtctgactgcagctggaacttctccactgtccctcctcccgagggcagctctccaaacacggccctggtcaccgaagccatagggaaagtttggcgtgtgcagccactgcccgctcttcaaactccagcgctcgctaagctagaggcgacccaagtttacaggagaaggggcgtgactcggctcagactcctccctttccctgcctggatttagggagtgaccgttcctgcaaaaaatagcccctggggcctttctaaatcaatcatttgcctgagggtaacaagaggggcaaactttgcagccacacttgtacttttttt

SEQ ID NO: 13983 - RNA, 8226 nt, Homo sapiens
  source 1..8226: mol_type = other RNA
gctgggattacaggcatgagccaccgcacacaggcctcctttttatttttatttttttaaagatttatttttactcttttcttcttatataatatgtatttcctcttatgttctttctagtttagtcttagtacccaaaaacatttttatatctttactgagatatggttcaaattagatacaattcatctacttaaaatgtacaattcaacatttttaggtatattcataagtatgtgcaaccataaccacagtaaacttcagaatattttagcatttcaaaaacaccctcccaaccctttagttattatcccctattcctgtatcccctgaacagccacttaattactttatgtctcatagattttcctgttctagacatttcataggaatagaatcactgctgataaagacatacccaagaaattaagccaagaaaaagaggtttaattggacttatagttccacatggctggggaggcctcagaatcatggcggtaggttaaaaatacttcttacagggtggcagcaagagaaatgagtaagatgcaaaagcggaaccccctgatgaaaccatcagatctcatgagacttattctctaccatgagaacagtatgggggaaaccacccccatgattcaaattatctcccaccaggtcccacgtataacacatgggaattatgggagtataattcaagatgaaatttgggtggggacacagagccaaaccatatcatcccacccctggctcctccaaatcttatgtcctcacatttcaaaaccaatcatgcattcccaacagtaccccaaagtcttaaatcatttcagcattaacccaaaagtccacagttcaaaagtctcatctgagacaaggcaagtcccttccacttatgagcctgtaaaatcaaaagcaagctagttacttcctagatacaatgagggtacaggtattgggtaaatacagccattccaaatgggagaaattggccaaaacaaaggggttacagggcccatggaagtccaaaatccagtggggcagtcaaattttaaagctccaaaatgatctccttttactccaggtctcacatccaggtcacgctgatgcaagaggtggcttcccatggtcttgggcagctctggccctgtggctttcagggtacagcctccatcctggctgctttcatgggctggtgttgagtatctgcagcttttccaggcacctggtacaagctgtaagtcgatctaccattctggggtctggaggacagtggtcctcttctcacagctccactaggcggtgtcccagtagggactctgtgagggggctccaaccccacatttcccttctgcactgccctagccgaggttctccatgagagccccgcccctgcagcaaacttctgcctgggcatccaggcatttccatacatcttctgaaatctagacagaggttcccaaaccccatttcttgacttctgtgcacccacatgctcaacatcacatggaagttgccaaggcttaaggctttcaccctctgaagccatggcctgagcttcatgttggcccctttcagccatggccggagtggctaggaaacagggcaccaagtccttagactgcacacagcacaaggaccctaggccttgcccacaaaaccatttttaccattttttcttcctagacctccaggtctgtgatagaagaggctgccacaaatgtctctgacatgccctggagacattttccccattgtcttggaaattaacattcagttccttgttacttatgcaaatatctacagccagcttgaatttctcctcagaaaataggattttcttttctatcgcattgtcaagctgctaattttctgaattttaatgctctgcttcccttttaaaactgaatgcctttaacaacacttgagtcacctcttgaatgctttgctgcttagaaatttcttccaccagatacccttaatcatctctctcaagttcagagttccacaaatctccagggcaggggcaaaatgccgccagtctctttgctaaatcataacaagagtcacctttgctccagttctcaacaggttcctcatctccacctgagaccacctcagtctagatttcattgtccatatcattatcagtatttttgtcaaagccattcaacaagtctcaaggaagttccaaactttcccattttcctgtcttcttctgagccctccaaactgttccaatctctgcctgttaccaagttccaaagttgcttccacatttcccggtatctttgcagcaacacctgctctactggtaccaatttactgtattagtccattttcacgctgctgataaaagacgtacctgagactggggaaaaaaaggggtttaattggacttacagttccacatggctggggaggcctcagaatcatggcaggaggtgaaaggcacttcttacatggcggccgcaagagaaaatgagtaagatgcaaaagcggaaacccctgataaaaccaccaggtcttgtgagagttattcactaccatgagaacagtatgagggaaactgcccccatgattcaaattatctcccactgggttcctcccacaacacatgggaattatgagagtacaattcaagatgagatttgggtggtgacacagagccaaaccatatcaggatgtttgggttgtttccacattttaactctacgtgtaatgctgcacccaagataatgcttccattccatgaatgggggatatgcatcaaaagagaactttaacaaagaaagtaaactcatttttgaattttaagatcactttggcattctgttttgaggtctgctaaacttgcaatgctgggtgaaaatgacttcaaaataaaaccaatgttgaaagacaccaagagactgtaactacttgagattccatttttcctttataatttatttgccacaatgttaaatactgtagatcatacagaatctgttttttctgcccaaaaatgggggtctgttatcaacagactcagccccaacctcgttcaggacaagcttgtgtggttcagaaggtagatcacagagcaggttgtacccatgcctttgccagcataatgaagttgactcttttggggtgggtgtcaaagctcctctcatgttctgttacattaaggtaaaaactgagggcccatagcaagggcccctatctagacaaaacctaatcatcttatcttggacaaatttctctgttctttctatagcctgtggtagacacaatgtgcccatcaaagatgtcaacacccaaatgcctgcaacctttgaatatattatataggaaaagggactttacagctataattaaaattatagatttttaaaataggaagattaccctggatatctggataggtccaatctaaccacatgagatcttaaaagcagtgaactcttgctagggcaagaaagatatggcagaaagggaattcagagagattgaaagcataagattcatctaccaatgctgaagaagcccacaagggaattcagagagactgaaagcatgagattcatccactaatgctgaagagggccacacagaaagtatgagaaggaatgtgggcaaattctagaaacaaagactagcccacagctaacagctagcaaggaaatggggaactcagtcctacaactgcaaggaactgaaatctacctaatgaggctgaaagaactcttatctagggacttccccttacagcctctagctaagagcccagctcagctgacaatctgattacagccttgtgaggctttaagcagaggacccagttgagccatattgtgcctagatttctgtgccatggaactgtgagataataaatgggtgttgttttaagctactaagtttgtagtaatttgatctagcagcaatagaaaattaataaacttttttttaaaaaaagcagaatttgcaagcaaatgtgactttgagcgtaattcttcttcactgcaaatatgtgatgtaggagtctttgagttatttgcttgagaataacagtgataaactatactcctatctgtgctcctcagtatttggttgcattcattggaagactgaggctctacttaggggattttttcctccaagtccttctagaataccctggaatggagaatgaattttaggagatcaggactgcagcatgaagatgaattatcaagctactgtactaatccagctgagggatgataggacagggttagctggtatggaagagtcagactggagaaggggacattgatgttgattcctaatagttctagaatggcttactaggtggatggtggggtggtatgcaggaagtaaatggatattgaaaactgaagctcagctgattctcaaattagtcactcccatttgggaattaacatgtaagttgataaaatcatgtcagtggagattacccaggagacacttatggatttgttttaaaatataaacaaaatataaatataacaaaatataataaaatataacaaaatataaacaaaatataaataaaatataaacaaaaatataaaacataaaaggaggaatgaggaagcattacatatagcgactaataggagattctgttgcttgggaaaggagagagaaaaaagaagaggcttagaaaagatgagaaagatgttggctaagttagatttgatacatcgcaaatgaactaaaaaaaagtggtaaatagtctctttttatattagtctattttcacactgctataaagaactacctgagactgggtaatttatgaagaaaagaggtttaattgactcacagttctgcatggctggggaggcctcaggaaatgtacaattatggtagaaagcaaagaagaagcaaggaccttcttcataatacagcaggaggtggggaggaagtgccacacttttaaaccatcagatctcatgagaactcacttaccatcatgagaacagcatgggggcaatcactcccatgatccaatcacctcccaccaagaccctccctcgacatgtgggaattacaatttgagaggagatttgggtgaggacacagagccaaatcacctcacccttagatggaaaaaaataagtagggggaaggcatgaagctagaaaaagttcttgttacctaccagggaacagtaccagtccaggacagctagattcctgtctttgtgaataatgatgatggtggaattggctacagaagacagaggcacaggaaaaagtgatagtgttcaaccagccatttgcacataggaagcttcacaagctgggcgtctgtaatttggggaatattaatattgtgttcctcttgagtatattattcattcagcaaagatttagctgtttacaaaatcatttacagagaaattggagactctttcaatcccctatttctgtgaaaacattgcagctgtactaagactgaaaaatcctagttagcttatacagtagctacctatgcattcaacagtttcctcacgaaaagctcacaatgactatccttgataccctttgctgatctgaatctgtgaaagtatttgacagttgcacaaagcagcaggaagagaaaataagttgcccacatgcaagaacctaagagggcttcctgctgaaccaccagttgtggagaaagcagccaaccaggggaagaaccattcaaggcagaatgttcctcatttttccagctgatttagatggactaaagaattaaaattcaacccattccaaagcaccaaataataactttatgctgtggaactagacactatactttcactctctttcctaatgtctttgtttttggctaagagtaaaaatagctgtcaaggttccctctctcaagctctgttaacacacctagtccaaaggcgcatgtgtgtcatgtctctaatatattttattgctgccttttaaaattccccttgagacgctggcccaatattgttgcattcaaccacatttctaccacaaggattaaaaagaacttaagtataattttattctattctgcatcaatgccatacacacacaaaaaaatgtttggatcacttaataagttataacattctatgttttaacattaataacaaggacataaatgatcatttcctgagttaacagtgcaaggtaaaatttaatctgtattgctaataagacattttacagcatagaaacatgatcgaagtgatcatttactttatcatgtcataaaacacaagtgcttattgtagaacagtgatataatttaaatggcaaggaaatttgtgattcataacaaagaatcctgtatgtatttgttgccatgattaactttccaggtcaaatatcagtagtaaaataagttgtggtacaaaagaaagccaagaagttacctgtactgaaggaacatttgatttcatttaagaaactgaaggctggattctagttaaccttttgttatgtacaaaaatgttctcttaaaaaaccctaagcaatcacaaatttagataaactagttgaataaaggacaatgacagctcttcattatgctgtaaaactatggatctcatttttggaaaagttgagatcatgcagcaaccttactccttgttctgtaaatggcactggtccacaaatgcagacgagaactttggatttgtccaaatttcttttcaaaaattcagaaagaagagctggtgaaatatgtccctgtttgccattccattcagaaataggtgctgagagaacaaattcaacatccagtcttttatctttaaatgctaatttctccaattggcttctccaaattatatcatcttctgttttattgaagaacatcagcttcactttcctgagactgggtatatcagtcaaagcataattcagtattttaaccattggtgtgaagcctgttccagctgccaacaaaaagagatcttctaattcttggaacttggatattttaaaattgccctcaggactgcttacagaaacaaaatctccaatctgaagacgatcaagctctggtgtgaagagtccagtgggatagatttttatcaaaaagtagatgtatttattgttgggaagaactggttccttgaactctgagagtaaggaaccagatacaggtgtatatggctttactatttctgtacctgtaataggtagcttgaggtaaacatgttgcccaatgggcacttgaagatgagtgcttggtggcagcatcaaacagaaaagcctcgtatcatgagtaacatcttccttggaaattaactggcactttctgtagtacaaacctgtatctttccttggaataagtgaattatgattcttcaggggatggccaagaaagtcccaagaagtattctcttttttttgtagaacaatctctatttttcccacactctcaacaacccgcacagaaaaatcttcctgaacctcatggcttagcccaatatgtataagatataaacaatccttaataattgtttctgctctaaaggaatcattctgatgatcaactattattgagtctaaattgatatccttctgtttagtatatatggcaatggtgactaaagagtctgtttggaaccaatcatagcttggataactaggaccttctttggcaagtgtatctgtcacttggctcttgggaagcatgccatttaagactttcttttcctcctcacgatagtctttcagaacagcaggtttaatggccattctgccaaccaggcattctttcagcatggattcataattgacccaacgatgaacctgatcaaaaagttcagtaccatctgatcctgctgctctcattagttcatcttctccaccaggatgatactccatataagggctgacattataaacgaaacctcttatgcatatccaacaatcatcttttttgttgtgtttcttaagttcttcttcagttacttcaattaacctgccttttaatcccgttagatcctttccacttttggtcagtcgaatccaatccataaggcttctgccctgttttaaaggtaccttgctacgccccccggaggcgacacgctgctgcgacctgggggccgggaaagactgggaagggacgttcagcatcttcaaaccccggccccgggccctgcccggggatcgccgccagacgggacagcacctccagctccggctctgtggccgggcagaggccaagccc

SEQ ID NO: 13984 - RNA, 4402 nt, Homo sapiens
  source 1..4402: mol_type = other RNA
gctgggattacaggcatgagccaccgcacccagaaaaagcaaatctcttagtatttttcctcttgtccaaaggttctgaccatgttcatgacctaagcttgtccctggaagcatacatgtccctgggagacaggaaggttcagggaacttctccaccctgattctagccaatggccagcgaactccttttccagggttggcttggcagtgtcggggaatgatgcaggttcatcgggatgggcatgaaaagaaagggaatggaagaggctgggaaagaacttgtggccatccctttcagaacagcatggagctctgaggacttagtattacagaaggtgaagtgttattaagtacatgagtgacatccggaccttgtggactaagaggacccctaaccaagggtcagcggggaactctgtggcacacaagtgtggcatttctggaagctcttgattgccttctggtcctgcctctgctgctaccctgatgagatctgagtttgttctgctggtggggtattctaaaatgtgggacgtagagctggagtccacgacatctatctggagactcatgtcaaatgtcctgtcattggcactacctcacttcctttgttgtttccttcctccagccagccctacctccatctcccacctgtctgcccagctctccctgaaggtcccttaccagcctcgactgggagacaagtccaccttttccagtctcaggctcttgcactcaccagaagaaccttttgtgattgcaaggtctgaaggggaagccagggatagagtcctgcaggaagctaacgggggtggaagtgggaaatggagtgaggctggggtgatctgagagggcttccttctggtttagatgggttcctgcttttggatgctgatctattacagtaggaagtggggttgaagggatgggagtgggcagggtggggtaacccttaattcctcagaaaaaatagacaacatagtggagtgggatggaaaaggatctggtcggggggactctaacacatagtgtctaatctgattgttcacagttaggtctatggggtcatcaccccaatttatataccccgcaacttagcctgctgagttgcctcattatctctccccaaatgttgccacccaatgccacccgttatttccatccctctccatcaccatccccacaacacctccagagctccccatctttccatgcctggttcttcttccaatggggtcagtagtatgtctccttctccacccagccaccaggataccgccgcaggatgagctttcggacctcatcatagatgaagatgaggaggctgtaggggaaggcgcagaaccaccaggtgactttgagcgggtacatgcggagggctacacccatgcctgggcagtaagagagaaaggcagccaacgccgtctcctccaggagcccaaaaatcaggatcttgttcttcatgccctgctggaagactgagttgcggcgggtcttgcagatgatgaggtcagcccactgcaccaccacgatgctggcaaagaatgccgtgtggcacgtgaactccaccaccttccgctgctcataggtccactcctgtccatagctgtcctccagatcattcatggtccggtcatcccagtcgaggcggattcccagtagccgtgatggcaggaaaccgttctctgccaggatcacaaagtaggtgaagaagccacccagtgcctggatcatcccgatctgtccgtaggccatgctgatgagcctctcattcaccagcttgtccgtctgggagtttcgtggctgccgcttcatgatatcactctcagctgcctcataggccaaggagatggcagggaccatatctgtgcccaggtcaatgcaaaggatggtcacagtgcccagaggtagggggatgttggcaatgatgaacagcaggaagggggtgatctcggggatgttgctggtcagggtgtaggcgatggatttcttcaagttgtcaaagatcaggcggccctcctccacccccgtgacgatggaggcaaagttgtcatccagcaggatcatgtcggctgcctgcttagagacgtcagagccagagatgcccatggcaatgccaatgtcagccttcttcaatgcaggggagtcgttcaccccgtcacccgtcacggccacaatggctccctgcctctgacatccctccacaatgatgagcttctgctggggagacgttcgagcaaagacgatctctgtgtggttcttgaggatctcatcgagctgctccgatgtcatgtccttcaggtcagagccgtgcaccacgcatgccttggcttctctggggttgacttgactcatgggaatgttgagccgggctgcaatgtcctccacagtctcgttaccctctgatatgatgcccacgcctttggcaatggccttggctgtgatagggtgatccccggttaccatgatcaccttgatgcctgcgcttcggcacttgcccacagcatctggcacagcagcccggggagggtcaatcatagacatgagccccacaaagcaaagcttctccgtgggaaagttcagctcatccgtgtcgaatttgaagccccgaggaaactttccagatggcagattcagttgacagaatcccagcacacgctccccaagtccccccagctccatgtaggcattttgaaaggcatcttgcatctccttgtcgagcgggatctccttgccctgcaccaggatggtggagcaccggtccagaatgcgctctggggcccccttcatcaccagcacgtggctctgggggctgtcttctcgctcgtggatagacagctggtacttgttggtagagttgaaaggaatctctgccaccttggggtttctgtctctcattttcctcactgagccacaggagagctcaatgcacttgagcagagctgactcagaggcatcaccagctgtgtcccgcttagacacggagatgttctcctgtcctgccttgaagacggcgcggttgcagagaccagcaattcgagacagggccgtccacgtaggggatcgtttgtcaaaagtggccccagactgatcttcggtggtgtcagcctcatggatttggttgtcgaaccacatgtgggcgacggtcatgcggttctgggtgagggtgcccgtcttgtccgagcagatggtggacgtggagcccagcgtctccaccgcctccaggttcttcaccaggcagttcttccgtgccatgcgcttggctgtcagggtcaggcacacagtgacagtggccagaagcccctcaggcacgttggccactatgatgccgatgaggaagatgactgcctccagccagctgtagcccaggatgagggagagcacgaagaaggagacccccaggaatacagcgacccctgtgatcagctggatgaagtgttcaatctccattgctatgggtgtccgcccaacctccaggcctgaggcgagagtagctatgcggcccatcaccgtccggtctcctgtggcaatcacaatgcccctggcagtgccttcaacacagttggtggagaagaaacagatattgcgggtctccagggggttctcatgggtgaactcgggggagcgggtctggggctccgactctcctgttaaggatgagttatccaccttacagccatgagaagagatgatccggaggtcagcagggacgcggtctccacccttcacctccaccaggtctcccaccaccacttcctctgcgttgatctgcatcttctctccctcccggatcacaagggcttgctgaggtaccatgttcttgaaggaatccatgatcttggagctcttggcctcctggtagtaggagaagcagccagtgacaatgaccacagctgccagcaccacacccagatatagattgtcgttggatggttcatcctccatggcagcctggatgccgtaggccaggaagcagaggatagccccaatccacagcaggatggagaaccccccgaaaagctgacggcagaacttgacccactcaggggttgtgggaggtggtgtgagggcgttgggcccatctcgagccagaacgtcctgagcccgctggttggtgaggcccttggacaggtccacttggtatttgcggcccagctcatccaaggacagcttgtggtcatccattgccacctccttcttcagctcatccagttccttctccttctgtttcttcttgccgcccccattctctgccgtggtggcggcaggtgagtactcacggccagccccacggcccatcttggggcagagtggctgagggaccttagcgggagaggtcaccaggaggatcccaagcccacaccagcccgtctgggacagtcggagaccctggcagacagag

SEQ ID NO: 13985 - RNA, 1283 nt, Homo sapiens
  source 1..1283: mol_type = other RNA
gctgggattacaggcatgagccaccgcacccagacgaaagagtgattttaaattttcctcttcaagggaaggtataaatgccaacctcatgaaaggtcaggacttaggatccaggcccaggaccacaggagatgggttcttaggaggctttagaaatttgctctgaaggaaaactcttggcacacacaggccttcttttttattcaccgtctctcgaaacacatactcgtttaccacttcttcataacctgtgtccataaagagctgagccaggaagtcatcagtaaaaaaatatgatctggtcccatcttgtctaacataaaagttttctccaagtttgctgctggctttaaacctaagcatggcatgatcatacagtccgtagtcacgaaacaagacacttttgcctggttttaataccttatagcaggactccatggatcccaggtaactgcaaaatcatccttgtcccagggctggcgaagctctgaagagcagccatggcacttgtaaatgttttgtaagacaaggtgcatcttatcaggatgaacagctgacagcacaaatatcaacataacaacatccacagactctggcggtacatgatccagaagatcatctttagtcagatcacactggaataccttgcatctttctgtatcatataaaggattttgcttaacatattcaatggctcttggagaaaaatcacaggcataggcaaagatattcggatcttcttctaaaagtgggaataaacagtttccaaccccacagccagcttcaagcattgttaacttttgatcttcaaactctctacatgatcttagctcctcaaactctctggtggtccagtgtctgtctttgaagaaattagtgctatttcttttgtaaaaaagatcccaatttttctgagcctcttgttccaatttctgctgtttaaaatcagacaccaaagtttggtctcttttcagtttctcctcttcttcagaggtgagaatccttgcctgcagccctttcctttgcaaagaagccatctctgaaactgacggtaacacttaacacagctgaagattctccatcaccaaataatatgaatccacgctaatggatcagatacatttcctgaggtgagtttcacgcctcaaacagcacagggggcccacagccagccccactgggcctcggaggcagaatacgggaagaaccgcgaaacaaccctaaaccaattctgaggaccacgaattcggattatccgggagttcttttgccatggcaccgcc

SEQ ID NO: 13986 - RNA, 1083 nt, Homo sapiens
  source 1..1083: mol_type = other RNA
gctgggattacaggcatgagccaccgcacccagacgaaagagtgattttaaattttcctcttcaagggaaggtataaatgccaacctcatgaaaggtcaggacttaggatccaggcccaggaccacaggagatgggttcttaggaggctttagaaatttgctctgaaggaaaactcttggcacacacaggccttcttttttattcaccgtctctcgaaacacatactcgtttaccacttcttcataacctgtgtccataaagagctgagccaggaagtcatcagtaaaaaaatatgatctggtcccatcttgtctaacataaaagttttctccaagtttgctgctggctttaaacctaagcatggcatgatcatacagtccgtagtcacgaaacaagacacttttgcctggttttaataccttgtaaatgttttgtaagacaaggtgcatcttatcaggatgaacagctgacagcacaaatatcaacataacaacatccacagactctggcggtacatgatccagaagatcatctttagtcagatcacactggaataccttgcatctttctgtatcatataaaggattttgctctctacatgatcttagctcctcaaactctctggtggtccagtgtctgtctttgaagaaattagtgctatttcttttgtaaaaaagatcccaatttttctgagcctcttgttccaatttctgctgtttaaaatcagacaccaaagtttggtctcttttcagtttctcctcttcttcagaggtgagaatccttgcctgcagccctttcctttgcaaagaagccatctctgaaactgacggtaacacttaacacagctgaagattctccatcaccaaataatatgaatccacgctaatggatcagatacatttcctgaggtgagtttcacgcctcaaacagcacagggggcccacagccagccccactgggcctcggaggcagaatacgggaagaaccgcgaaacaaccctaaaccaattctgaggaccacgaattcggattatccgggagttcttttgccatggcaccgcccccgccacttccgctaggaac

SEQ ID NO: 13987 - RNA, 1218 nt, Homo sapiens
  source 1..1218: mol_type = other RNA
gctgggattacaggcatgagccaccgcacccagacgaaagagtgattttaaattttcctcttcaagggaaggtataaatgccaacctcatgaaaggtcaggacttaggatccaggcccaggaccacaggagatgggttcttaggaggctttagaaatttgctctgaaggaaaactcttggcacacacaggccttcttttttattcaccgtctctcgaaacacatactcgtttaccacttcttcataacctgtgtccataaagagctgagccaggaagtcatcagtaaaaaaatatgatctggtcccatcttgtctaacataaaagttttctccaagtttgctgctggctttaaacctaagcatggcatgatcatacagtccgtagtcacgaaacaagacacttttgcctggttttaataccttgtaaatgttttgtaagacaaggtgcatcttatcaggatgaacagctgacagcacaaatatcaacataacaacatccacagactctggcggtacatgatccagaagatcatctttagtcagatcacactggaataccttgcatctttctgtatcatataaaggattttgcttaacatattcaatggctcttggagaaaaatcacaggcataggcaaagatattcggatcttcttctaaaagtgggaataaacagtttccaaccccacagccagcttcaagcattgttaacttttgatcttcaaactctctacatgatcttagctcctcaaactctctggtggtccagtgtctgtctttgaagaaattagtgctatttcttttgtaaaaaagatcccaatttttctgagcctcttgttccaatttctgctgtttaaaatcagacaccaaagtttggtctcttttcagtttctcctcttcttcagaggtgagaatccttgcctgcagccctttcctttgcaaagaagccatctctgaaactgacggtaacacttaacacagctgaagattctccatcaccaaataatatgaatccacgctaatggatcagatacatttcctgaggtgagtttcacgcctcaaacagcacagggggcccacagccagccccactgggcctcggaggcagaatacgggaagaaccgcgaaacaaccctaaaccaattctgaggaccacgaattcggattatccgggagttcttttgccatggcaccgcccccgccacttccgctaggaac

SEQ ID NO: 13988 - RNA, 1097 nt, Homo sapiens
  source 1..1097: mol_type = other RNA
gctgggattacaggcatgagccaccgcacccagacgaaagagtgattttaaattttcctcttcaagggaaggtataaatgccaacctcatgaaaggtcaggacttaggatccaggcccaggaccacaggagatgggttcttaggaggctttagaaatttgctctgaaggaaaactcttggcacacacaggccttcttttttattcaccgtctctcgaaacacatactcgtttaccacttcttcataacctgtgtccataaagagctgagccaggaagtcatcagtaaaaaaatatgatctggtcccatcttgtctaacataaaagttttctccaagtttgctgctggctttaaacctaagcatggcatgatcatacagtccgtagtcacgaaacaagacacttttgcctggttttaataccttgtaaatgttttgtaagacaaggtgcatcttatcaggatgaacagctgacagcacaaatatcaacataacaacatccacagactctggcggtacatgatccagaagatcatctttagtcagatcacactggaataccttgcatctttctgtatcatataaaggattttgcttaacatattcaatggctcttggagaaaaatcacaggcataggcaaagatattcggatcttcttctaaaagtgggaataaacagtttccaaccccacagccagcttcaagcattgttaacttttgatcttcaaactctctacatgatcttagctcctcaaactctctggtggtccagtgtctgtctttgaagaaattagtgctatttcttttgtaaaaaagatcccaatttttctgagcctcttgttccaatttctgctgtttaaaatcagacaccaaagtttggtctcttttcagtttctcctcttcttcagaggtgagaatccttgcctgcagccctttcctttgcaaagaagccatctctgaaactgacggtaacacttaacacagctgaagattctccatcaccaaataatatgaatccacgctaatggatcagatacatttcctgaggtgagtttcacgcctcaaacagcacagggggccgacgccggaagtcccacggc

SEQ ID NO: 13989 - RNA, 1097 nt, Homo sapiens
  source 1..1097: mol_type = other RNA
gctgggattacaggcatgagccaccgcacccagacgaaagagtgattttaaattttcctcttcaagggaaggtataaatgccaacctcatgaaaggtcaggacttaggatccaggcccaggaccacaggagatgggttcttaggaggctttagaaatttgctctgaaggaaaactcttggcacacacaggccttcttttttattcaccgtctctcgaaacacatactcgtttaccacttcttcataacctgtgtccataaagagctgagccaggaagtcatcagtaaaaaaatatgatctggtcccatcttgtctaacataaaagttttctccaagtttgctgctggctttaaacctaagcatggcatgatcatacagtccgtagtcacgaaacaagacacttttgcctggttttaataccttgtaaatgttttgtaagacaaggtgcatcttatcaggatgaacagctgacagcacaaatatcaacataacaacatccacagactctggcggtacatgatccagaagatcatctttagtcagatcacactggaataccttgcatctttctgtatcatataaaggattttgcttaacatattcaatggctcttggagaaaaatcacaggcataggcaaagatattcggatcttcttctaaaagtgggaataaacagtttccaaccccacagccagcttcaagcattgttaacttttgatcttcaaactctctacatgatcttagctcctcaaactctctggtggtccagtgtctgtctttgaagaaattagtgctatttcttttgtaaaaaagatcccaatttttctgagcctcttgttccaatttctgctgtttaaaatcagacaccaaagtttggtctcttttcagtttctcctcttcttcagaggtgagaatccttgcctgcagccctttcctttgcaaagaagccatctctgaaactgacggtaacacttaacacagctgaagattctccatcaccaaataatatgaatccacgctaatggatcagatacatttcctgaggtgagtttcacgcctcaaacagcacagggggcgtcatcagttcctaaattcac

SEQ ID NO: 13990 - RNA, 1141 nt, Homo sapiens
  source 1..1141: mol_type = other RNA
gctgggattacaggcatgagccaccgcacccagacgaaagagtgattttaaattttcctcttcaagggaaggtataaatgccaacctcatgaaaggtcaggacttaggatccaggcccaggaccacaggagatgggttcttaggaggctttagaaatttgctctgaaggaaaactcttggcacacacaggccttcttttttattcaccgtctctcgaaacacatactcgtttaccacttcttcataacctgtgtccataaagagctgagccaggaagtcttatagcaggactccatggatcccaggtaactgcaaaatcatccttgtcccagggctggcgaagctctgaagagcagccatggcacttgtaaatgttttgtaagacaaggtgcatcttatcaggatgaacagctgacagcacaaatatcaacataacaacatccacagactctggcggtacatgatccagaagatcatctttagtcagatcacactggaataccttgcatctttctgtatcatataaaggattttgcttaacatattcaatggctcttggagaaaaatcacaggcataggcaaagatattcggatcttcttctaaaagtgggaataaacagtttccaaccccacagccagcttcaagcattgttaacttttgatcttcaaactctctacatgatcttagctcctcaaactctctggtggtccagtgtctgtctttgaagaaattagtgctatttcttttgtaaaaaagatcccaatttttctgagcctcttgttccaatttctgctgtttaaaatcagacaccaaagtttggtctcttttcagtttctcctcttcttcagaggtgagaatccttgcctgcagccctttcctttgcaaagaagccatctctgaaactgacggtaacacttaacacagctgaagattctccatcaccaaataatatgaatccacgctaatggatcagatacatttcctgaggtgagtttcacgcctcaaacagcacagggggcccacagccagccccactgggcctcggaggcagaatacgggaagaaccgcgaaacaaccctaaaccaattctgaggaccacgaattcggattatccgggagttcttttgccatggcaccgcc

SEQ ID NO: 13991 - RNA, 1055 nt, Homo sapiens
  source 1..1055: mol_type = other RNA
gctgggattacaggcatgagccaccgcacccagacgaaagagtgattttaaattttcctcttcaagggaaggtataaatgccaacctcatgaaaggtcaggacttaggatccaggcccaggaccacaggagatgggttcttaggaggctttagaaatttgctctgaaggaaaactcttggcacacacaggccttcttttttattcaccgtctctcgaaacacatactcgtttaccacttcttcataacctgtgtccataaagagctgagccaggaagtcttgtaaatgttttgtaagacaaggtgcatcttatcaggatgaacagctgacagcacaaatatcaacataacaacatccacagactctggcggtacatgatccagaagatcatctttagtcagatcacactggaataccttgcatctttctgtatcatataaaggattttgcttaacatattcaatggctcttggagaaaaatcacaggcataggcaaagatattcggatcttcttctaaaagtgggaataaacagtttccaaccccacagccagcttcaagcattgttaacttttgatcttcaaactctctacatgatcttagctcctcaaactctctggtggtccagtgtctgtctttgaagaaattagtgctatttcttttgtaaaaaagatcccaatttttctgagcctcttgttccaatttctgctgtttaaaatcagacaccaaagtttggtctcttttcagtttctcctcttcttcagaggtgagaatccttgcctgcagccctttcctttgcaaagaagccatctctgaaactgacggtaacacttaacacagctgaagattctccatcaccaaataatatgaatccacgctaatggatcagatacatttcctgaggtgagtttcacgcctcaaacagcacagggggcccacagccagccccactgggcctcggaggcagaatacgggaagaaccgcgaaacaaccctaaaccaattctgaggaccacgaattcggattatccgggagttcttttgccatggcaccgcc

SEQ ID NO: 13992 - RNA, 1104 nt, Homo sapiens
  source 1..1104: mol_type = other RNA
gctgggattacaggcatgagccaccgcacccagacgaaagagtgattttaaattttcctcttcaagggaaggtataaatgccaacctcatgaaaggtcaggacttaggatccaggcccaggaccacaggagatgggttcttaggaggctttagaaatttgctctgaaggaaaactcttggcacacacaggccttcttttttattcaccgtctctcgaaacacatactcgtttaccacttcttcataacctgtgtccataaagagctgagccaggaagtcttgtaaatgttttgtaagacaaggtgcatcttatcaggatgaacagctgacagcacaaatatcaacataacaacatccacagactctggcggtacatgatccagaagatcatctttagtcagatcacactggaataccttgcatctttctgtatcatataaaggattttgcttaacatattcaatggctcttggagaaaaatcacaggcataggcaaagatattcggatcttcttctaaaagtgggaataaacagtttccaaccccacagccagcttcaagcattgttaacttttgatcttcaaactctctacatgatcttagctcctcaaactctctggtggtccagtgtctgtctttgaagaaattagtgctatttcttttgtaaaaaagatcccaatttttctgagcctcttgttccaatttctgctgtttaaaatcagacaccaaagtttggtctcttttcagtttctcctcttcttcagaggtgagaatccttgcctgcagccctttcctttgcaaagaagccatctctgaaactgacggtaacacttaacacagctgaagattctccatcaccaaataatatgaatccacgctaatggatcagatacatttcctgaggtgagtttcacgcctcaaacagcacagggggctgcagggctagggccaggcgcactcaccccacagccagccccactgggcctcggaggcagaatacgggaagaaccgcgaaacaaccctaaaccaattctgaggaccacgaattcggattatccgggagttcttttgccatggcaccgcccccgccacttccgctaggaac

SEQ ID NO: 13993 - RNA, 256 nt, Homo sapiens
  source 1..256: mol_type = other RNA
gctgggattacaggcatgagccaccgcacccagccagtcaattgatttttgatgaaagtaccaaggccatttaattgagaaatgacagtcttttcaacaaatgatgttggaacaattgggacacccatatgcaaaaaactgaacattgagtcataccttacatcttatacaaaaataattcaatacatcacagtcctaaacaaaaaacctaaaactataaattctaggagaagacaggagaaaattttataacctt

SEQ ID NO: 13994 - RNA, 1191 nt, Homo sapiens
  source 1..1191: mol_type = other RNA
gctgggattacaggcatgagccaccgcacccagcccaaatctccagtttctaaactggtaagctcaagttgctatgcctcaaggaatttgagagaatatttaatgtaagattcaggacccaatagtaagaattctactcaggacatctgatcttcattgaaacggattctaatccaacttcagtcctcatagcaaggaagtactatttcagaaagtccctagattctcagatgcattggcaagaaccatacactgaagaattcacagaagattttagtcacttgctcactcatccacttgaagtaagaaaaatcaatcactgcatgtttattgttactaaagggcattcttcggctacctctgccagcagatgagcggctccttgatctttgtgtttctaagatttgtcctagtccatttatggatctaattgtcgttcttaatttctttacatcttcttctggaaccaagtctgttttattaatgagaatgatatctgccaaagcaacttgcctagtagcttcattgataaggccatcaggtttctcttctgttaaatgttttaatccatattttgaatccacaatagttatgataccatcaaggtaaatatcactccctaattcagcatcaacccaaaacatagaagtcactgcaccagggtctgctaatccagtggtctctaacagtatgtcatcaaatttccccttcttttgcatcaaattctcaatagctctaaggccattgtccttcactgaacagcagaggcaaccgtttctaagttccagccactcttcatagagctctccaccttggctgacagctaaggatttctccagcgcacttccttccccagattcatttaaaatgaccgctactcttttactatgttgctctgtcaaaatatagttcagaagtgttgtcttcccagcacctaaatacccggtgataattgtgactgggatcttggcgccgaggccagacttttcctcctcctcgctttgcgtcgtctcaatgggaaccaattcaggacaatcctcctccgcaggatcctcttcctcatccacagatccaacagccggtaacattccggcctacggcacgtccctacctcagctgaaccgctgggaccaacacgccgtaccgcagccgcgcacgcccagcacgccactcccggcctggccggggcct

SEQ ID NO: 13995 - RNA, 1104 nt, Homo sapiens
  source 1..1104: mol_type = other RNA
gctgggattacaggcatgagccaccgcacccagcccaaatctccagtttctaaactggtaagctcaagttgctatgcctcaaggaatttgagagaatatttaatgtaagattcaggacccaatagtaagaattctactcaggacatctgatcttcattgaaacggattctaatccaacttcagtcctcatagcaaggaagtactatttcagaaagtccctagattctcagatgcattggcaagaaccatacactgaagaattcacagaagattttagtcacttgctcactcatccacttgaagtaagaaaaatcaatcactgcatgtttattgttactaaagggcattcttcggctacctctgccagcagatgagcggctccttgatctttgtgtttctaagatttgtcctagtccatttatggatctagtagcttcattgataaggccatcaggtttctcttctgttaaatgttttaatccatattttgaatccacaatagttatgataccatcaaggtaaatatcactccctaattcagcatcaacccaaaacatagaagtcactgcaccagggtctgctaatccagtggtctctaacagtatgtcatcaaatttccccttcttttgcatcaaattctcaatagctctaaggccattgtccttcactgaacagcagaggcaaccgtttctaagttccagccactcttcatagagctctccaccttggctgacagctaaggatttctccagcgcacttccttccccagattcatttaaaatgaccgctactcttttactatgttgctctgtcaaaatatagttcagaagtgttgtcttcccagcacctaaatacccggtgataattgtgactgggatcttggcgccgaggccagacttttcctcctcctcgctttgcgtcgtctcaatgggaaccaattcaggacaatcctcctccgcaggatcctcttcctcatccacagatccaacagccggtaacattccggcctacggcacgtccctacctcagctgaaccgctgggaccaacacgccgtaccgcagccgcgcacgcccagcacgccactcccggcctggccggggcct

SEQ ID NO: 13996 - RNA, 1762 nt, Homo sapiens
  source 1..1762: mol_type = other RNA
gctgggattacaggcatgagccaccgcacccagcccaaatctccagtttctaaactggtaagctcaagttgctatgcctcaaggaatttgagagaatatttaatgtaagattcaggacccaatagtaagaattctactcaggacatctgatcttcattgaaacggattctaatccaacttcagtcctcatagcaaggaagtactatttcagaaagtccctagattctcagatgcattggcaagaaccatacactgaagaattcacagaagattttagtcacttgctcactcatccacttgaagtaagaaaaatcaatcactgcatgtttattgttctataataaagcaaatgttagaaataaaagttagaaatgtcaaacacactaaattgttacataataaactaatcaagacacaacttttattcaggacatggatatttctgaaatgaaaacaaaagaagagaattgacttaaaatgtttataaatacgaatattatgacagaaccaaagctatttatgagcattatttttaaaagcttgtttaagtattatgcacttgtctgtgtgacattttgtaaagcggagaaaaattaaggagaaaggaattgtagaacactaacaggaagaggacagatactgaggaatggctcatggtataagtgagattatcagagactttctacaatggaatttgaaatgcagggagcacatttggtgtatggttgtagaggacttacactaaagggcattcttcggctacctctgccagcagatgagcggctcctgagaatgcataccaaattaattccccagctgttcacatgcatataagcagctgctgctgttactgcctaacacttaatggcagtctggcagcacctctaatctctgccatagcagacaagccactcatctaaggcctctgctgtacttccaaagaaagaatttctcaagtagagactgagtagaactagactgccagctgtgagcctcagagctcctggctgcctgttgctgagtctatcagctgctgagccttgatctttgtgtttctaagatttgtcctagtccatttatggatctagtagcttcattgataaggccatcaggtttctcttctgttaaatgttttaatccatattttgaatccacaatagttatgataccatcaaggtaaatatcactccctaattcagcatcaacccaaaacatagaagtcactgcaccagggtctgctaatccagtggtctctaacagtatgtcatcaaatttccccttcttttgcatcaaattctcaatagctctaaggccattgtccttcactgaacagcagaggcaaccgtttctaagttccagccactcttcatagagctctccaccttggctgacagctaaggatttctccagcgcacttccttccccagattcatttaaaatgaccgctactcttttactatgttgctctgtcaaaatatagttcagaagtgttgtcttcccagcacctaaatacccggtgataattgtgactgggatcttggcgccgaggccagacttttcctcctcctcgctttgcgtcgtctcaatgggaaccaattcaggacaatcctcctccgcaggatcctcttcctcatccacagatccaacagccggtaacattccggcctacggcacgtccctacctcagctgaaccgctgggaccaacacgccgtaccgcagccgcgcacgcccagcacgccactcccggcctggccggggcct

SEQ ID NO: 13997 - RNA, 1145 nt, Homo sapiens
  source 1..1145: mol_type = other RNA
gctgggattacaggcatgagccaccgcacccagcccaaatctccagtttctaaactggtaagctcaagttgctatgcctcaaggaatttgagagaatatttaatgtaagattcaggacccaatagtaagaattctactcaggacatctgatcttcattgaaacggattctaatccaacttcagtcctcatagcaaggaagtactatttcagaaagtccctagattctcagatgcattggcaagaaccatacactgaagaattcacagaagattttagtcacttgctcactcatccacttgaagtaagaaaaatcaatcactgcatgtttattgttcttgatctttgtgtttctaagatttgtcctagtccatttatggatctaattgtcgttcttaatttctttacatcttcttctggaaccaagtctgttttattaatgagaatgatatctgccaaagcaacttgcctagtagcttcattgataaggccatcaggtttctcttctgttaaatgttttaatccatattttgaatccacaatagttatgataccatcaaggtaaatatcactccctaattcagcatcaacccaaaacatagaagtcactgcaccagggtctgctaatccagtggtctctaacagtatgtcatcaaatttccccttcttttgcatcaaattctcaatagctctaaggccattgtccttcactgaacagcagaggcaaccgtttctaagttccagccactcttcatagagctctccaccttggctgacagctaaggatttctccagcgcacttccttccccagattcatttaaaatgaccgctactcttttactatgttgctctgtcaaaatatagttcagaagtgttgtcttcccagcacctaaatacccggtgataattgtgactgggatcttggcgccgaggccagacttttcctcctcctcgctttgcgtcgtctcaatgggaaccaattcaggacaatcctcctccgcaggatcctcttcctcatccacagatccaacagccggtaacattccggcctacggcacgtccctacctcagctgaaccgctgggaccaacacgccgtaccgcagccgcgcacgcccagcacgccactcccggcctggccggggcct

SEQ ID NO: 13998 - RNA, 1058 nt, Homo sapiens
  source 1..1058: mol_type = other RNA
gctgggattacaggcatgagccaccgcacccagcccaaatctccagtttctaaactggtaagctcaagttgctatgcctcaaggaatttgagagaatatttaatgtaagattcaggacccaatagtaagaattctactcaggacatctgatcttcattgaaacggattctaatccaacttcagtcctcatagcaaggaagtactatttcagaaagtccctagattctcagatgcattggcaagaaccatacactgaagaattcacagaagattttagtcacttgctcactcatccacttgaagtaagaaaaatcaatcactgcatgtttattgttcttgatctttgtgtttctaagatttgtcctagtccatttatggatctagtagcttcattgataaggccatcaggtttctcttctgttaaatgttttaatccatattttgaatccacaatagttatgataccatcaaggtaaatatcactccctaattcagcatcaacccaaaacatagaagtcactgcaccagggtctgctaatccagtggtctctaacagtatgtcatcaaatttccccttcttttgcatcaaattctcaatagctctaaggccattgtccttcactgaacagcagaggcaaccgtttctaagttccagccactcttcatagagctctccaccttggctgacagctaaggatttctccagcgcacttccttccccagattcatttaaaatgaccgctactcttttactatgttgctctgtcaaaatatagttcagaagtgttgtcttcccagcacctaaatacccggtgataattgtgactgggatcttggcgccgaggccagacttttcctcctcctcgctttgcgtcgtctcaatgggaaccaattcaggacaatcctcctccgcaggatcctcttcctcatccacagatccaacagccggtaacattccggcctacggcacgtccctacctcagctgaaccgctgggaccaacacgccgtaccgcagccgcgcacgcccagcacgccactcccggcctggccggggcct

SEQ ID NO: 13999 - RNA, 11652 nt, Homo sapiens
  source 1..11652: mol_type = other RNA
gctgggattacaggcatgagccaccgcacccagcccaatgtatatctttataaagctgggaccaaactggcttcttgcagcaataattaaatgttcaaatatgctcaacagaactttccctctagataatcatcatatctctaaatgtaatcacagttgtttgttttccaaactattacataaagagaacaatctcaaacttattgcattagcctttacacaagttatgttctttactaagtcactgaacacactgtacagttcagttgatatgctttttctaccaagactttttcaaataaaaagatatagtaggttgatttacattctagggcaagctccttaatttaggtaattattccggaatgttctcttaccactgctgctatccatccaattggattcctacaaagcttcaaaccacattaattaacaaagtaatttattccacactttactgttgtttagagttagctgtttgttggcaatgaagtggaaaaaagagaatcttccttcatattactatcatattcaaatagcatataaactaattgccatattagtaatatctatatattaatggtacatcaaaccaattgcaagaaaaggtaatttattagctttctttgttctatgggttgatcttcctggatatttcaaattgttgtgtgttggtaactggtaattgaagtactttctttgccacacagtctcccaacatttctaagaatctttgatgctgattattattaagacaattattgtctatatataagattattgtcttaattgcattttttagttttagcaatctaaagttgcttaaagatgtctaaaaagcattaacgtttatttgtgaaataatgaatatctgtgctttcagttttttaattacttaggtttttctttcaaagagatcttctggttttggatttatctctttatgttctgtatttaaatgttgatttagttttgattattttattgcttcatttgccagaacttctcagcaaataacatgttatggttttcccatgtcttcatttatggctaaaaaactgaactcagtatatgaagaattatatttatgagtaaaactagaacaatctattggttttcatttattcagaatcgcttttattgtcaccattaggtttactaatactgttgcattcagaaaaggtaagtcttttcttgataaaaaaagccagtgaagttattttgccatccataacatggtgttaaagataaatgaaacaaattaccccaaaccttcacatcgattgcattccctgcctgaaactttctctcctttctctttaaacagatctaatcttaacactggtcccccataaaaatatttccagtgcatatatctgacaaaagatttatccaaaatatttaaagaaatattataacttcaatcataagaagaaaaaataatgagtaaatagatgttccatatcacatattatcagggaaatgcaaattaaaataaatgtgatgtggatgagctgtctgagcagagaaaaacacaaaacaagtgagacaccactacacaccttttagaatggccaaaattcagaacactaacaccaagtgctgacagggatgttgagcaataggaacccttattcactgctggtgggaatgcaaaatggtacagcctctctgtaggacagtttggtggttttttacaaaacgaaacattctcttagcattcaatccaacaattgtgctctttggtatttacccaaaggagttgaaagcttaaatggacacaaaaacctacacatggatatctatagcaattttattcataattgccaaaacttggaagcaatcaaccaagatgtccttcagcaggtgaatggataaactgttgtacacccagacaatggagtattactcgatgctaaaaagaaatgagctatcaaactgtgaaaagacatagaggaaacaaatgcatattatccagtgaaagaaaccaatgtgaaaaggctatatatactttatgattccaactatatggcgttctgaaaaaggaaaaacttacggagacagtgaaaagaccagtggtagccgggggtcagtggggaggacacgacgaagaggcagagccaagggtttttaggacagtgtagactctgcatgactataaagatggatacatgtcattgtacctttgttcaaacccatagattgtacagcaccaagagtgaaccctaatggaaacaataggctttgggtgataatgatgtgtcagtgtaggtttatcaattgtaaccaatgtgccactctgctgggggatggtgatgagggaggcatgggggaggggagcactgaggatatataagttatttctgtaccctcctctcaattttgctcagaacctaaaactacttttaaaaactaaagttttttttttttttcaggagatgaggatctcactatgttgcccaggctgcagtgcagtggctattcacaggtgtgatcccactactgatcagcacaggagttttgacctgctccacttctgacgctccttaggcaactctgggtcccagtgacccaggaggtcactacatttatgctgaacttagtgcaaacacctgattgacatagctcactacaacccagaacttctggactcaagtgatcctcctgtcttagcctcctgagtagctaggtctacaggcatgtgccactgtgcctggcaaaaagtcttttttaagtgctaagaaaaaaaaaagagcaaatgatttgaacagatatttcaccaaagatatgagtgcccaacaagtacctgaatcaaaacttaatgttattgatcatcagagaaatgcaaattaaaaccatcaaattattactatatatccattagaatggctaaaactaaaaatattatcaaatgagggcaagaatatagcaattggaactttcattcatggtggtgagaatataaaatggtacaaccactttgcaaaaagcgttttggcagttttttttttttttttgagacggaatctcgttttatcacccagactggagtgcagtggtgtgatcttggcccactgcaacctctgcctcctgggttcaagggattctcctgcctcagcctcctgagtagctaggattacagatgcctgccaccacacccagctaatttttgcatttttagtagagacggggtttcaccatgttagctaggctggtctcaaactcctgacctcaagtgatccgcccacctccgcctcctaaagtgctgggattacaggtgtgaactaccacgcccagccccccagctcattcttagctaactagtgtgtgtgaaaaagagacagtgttaaaatatatatggtttaaactgataaggaaatgatcagttattgagcttatccatgattgctaattcaggtagagatggcttataagtaagtgttcggggctgcttacgggaagaaaaaatgaaagttagggatttcctttggatgctgggaaacaaaactccaactgggttctgacaaacataccatgtgcattgtcctgtggagacatgacaatgtaaacccataaacaaatcgattacgttttggtgacaactattgtgaagagaatggccatagtatttgctgcttctccttttaataggtagcatctctcctcttactcccttgaatctgagatagccttatgaagtgatattgtgccagttctgagactaggcctcaagaagcctcgaagcttccaatcttgcacttttttgtttgttttgatacaggtgcttgttctgttgcccagcctagagtgcagtggcacaatcatggctcactacagcctcaatctcatgggctcaagcaatcctcccatctcagcctcccaaatagctgggactacaggcatgcagcaccaccccaccctccccacccccagctaattttttaaaatttttttgtagaagaccaggcgtggtggctcacacctgtaatcccagcactttgggaggctgaggcaggcagatcacctgaggtggggaattcaagaccagcctgaccaacacggagaaacccatctctactaaaaatacaaaattagctgggcgtggtggctcatgcctgtaatctcagctactcaggagactgaggcaggagaatcgcttgaacccaagaggcaaaggttctggtgggctgagattgcgccattgcactccagcctgggcaacaagggcgaaactccatctcaaaaaatttttttttttacagatgggctctcactatgttgcccaggctggtcttgaactcctgggctcaagaaatcccccaaccttggcctcccaaagtgctgggattacaggtgtgagtcatcatgcccagccccaatctcatactcttgaaatcctaaagccatgtgaagaatccaggcctagcttgctggatgatgagagacacagtccccctaatgccccaggtgacagtcactcaataccagacatatgagtgacaccatctaggactagccagcctcaacaacccaactagtgacctcagctgcatgggcaagtccagccaagataagctgagctggatccagactataagaattacctggaagaacgcaaactaatgaaagattgttgttttaagccaatgagctttggggtgatttgttaattggcaatagataactgatattcaaggattcatccaaagttcccttaaaagatagaacccattaagtcattttaaacacttataagcaagttattaaatccttaaaagaaactgaaagtttctaaggtatactgggttggaaaaaggaaaagaaaaagaaactaaaagtgaaggctgaaactgacaagtaaggagttatttctccctgcaaatgtaatcagaaaataaggtggagtgtctctgaatgcataactggaacaaggaaacaatctaatggttttagtagtaaatatatgatttcaggggcacatccagtggaatgatggagtcagtgcacaacaacttgtaagacccagtcatggaaactggcaaacattacaagttagaaccagttgttaaatcttcattagtacatcactggacacatctattgctaaaggcacatttcatcagtatgtatatgcataaatatacatataagatgtccttaatgtttaaaaaagacattggttggttctgccacaatctgtgatcttgggcaagtcaattagtgtctttggatctgtttccaaatcagtccccaaaaatcatctttaagatgtctttcagctttacgattctatcttctatgctcttatggtaattacacctggatgcagcaattgaaaagtccaatgggatcaatccaaattgccacacttaaccatgttactgactacatatattactcatcaagacaattattcaagtaagtggcataatagtaatccaatgtactttgcattatgagtgaagaagagactaattttgactagaggggaaagaagggatggtcatagcaagatactttgtcaatcaggaatgagggctatctttgaacccacagtggcttgaactctataggtgcttaataaaatttgccgaaaagattacatgcttagagacaacattataaagaaaagacattcttggccgggcgtggtggctcatgcctgtaatcccagcacttcaggaggcgaaagcaggtggatcacctgaggtcaggagtttgagaccagcctgaccaacatggagaaaccccatctctactaaatacaaaaaattagccggacatggtgttgcatgcctatagtcccagctacttgggaagctgaggcaggagaatcgcttgaacccgggaggtggaggttgcagtgagctgagaatgtgccactacactccagccaaggcaacaagagcaagactctgtcccaaaaaaaaaaaaaaaaaaaaaagagacattcttgctgaattgaagactcagaagaggctgggcacagtggctcacccttgtaatcccagtattttggggggccaaggtgggcagatcacctgaggtcaggagttcaagaccagcctggccaacgtggtgaaaccccatctctactgaaaatacaaaaaatcagccaggcatgctggtgcacgctcataatcccagctactcgggaggctgaggcaggagaattgcttgagcctatgaggcggaggttgcagtgggctgagatcatgccactggccactgtactgcactccagcctgggtgacaaaagtgaaactccatctcaaaaaaaaaaaaaaaaaaaagactcagaagtaatcataaggttctacttgctattctcacatgtaattgtgagactctgcctccatttctccatctaaaaacaggagctcatttacaagcaacatgacaagaattcaagcagtcatggctgtgaagcatttctgcagaaggatatgctatgtaagtatgaggttgttactaaatcaaaatgaatgcctttgtgcaaaactagaaagcacattacatattgttcctgagtattccttcccagtgcattcaaaatattctcacattcacaaggttaaacagcacattaaaaaatagtaggaggctgatggctgagctcaattgggagtatctttctttggtgttagaatgtttgaaaattattttgggaagactatgagcaagttattttgaacttctggggaaaaaaaaaaatctgaagaagcattccctttgcctaaaagcaaaggagacatttatttatgcctttagcaaataaaatagtttgcttactaccagtgtttgtgggctgatattcaactcatcttctggaaattttaaaaatacacattgaaactgaaaaagtattctttgagtaagggtttacctgaagtgcccagaaccatccaaaatgatggcacattatatctttttttcttaaaaatttttggaatctaattgaagatgcctcttagaatatgtggaaaccacacgtgctatcttgcatatcactatcatttcagttctaatgttattaggtgtttagctacaggcaagtagaattagggcatgatgtgacagactgtaatgagttgctgagaaactacatactctatccccaggaaaacacatattctcaaaattctacacaatttcaggaatttcatagatgcccctaccccaaatcccattcatgaaatccttagcttaaaatcctgtgcactagagcaatgtattttataaaaccatattcagatgcctgtgaagcaatgaatgtgctaggcaatgttaggcggtagaaacagtgatacacgtagtcagacagggtacctagaagtcatggagcttataggctagtaggggatatggacatttaccaaataatcacacaaaaagatgcctaattacaaactctgattaagtgctatggagagatatacagtgttgcacgtaacaacagaatctaaagaagttacattttagggggcatataaacaatgttgtgcaggggaggtagaagaaacacattatggtaaagggctgcaaaggaaataagcccataataaggcctcttataggtttaagctaggacctgaaacttgtatactttatatgctttgaaatgagacatacattaaagtggctgatcaaattaaaacattttccagtctttgcctactaaattgataaagattttttaaaattttaatagaactaaagagaaaatatttctatatactgatgttaggagtatgcagtttaggccaggcatggaggctcacacctataatcccacccagcactttgggaggccaaggtgtgtggacacttgaggtcaggagttcgagaccagcctgaccaacatggtgaaaccctgtctctactaaaaatgcaaaattacctgagtatggtggtgcacacttgtaatcccaactacttaaggaggctgaggcaggagaatcacttgaacccgggaggtggaggctgcagtgagccaagatcgcgccattgcattccagcttgggcagagcaaacctccatctccaaaacccaaaaagtatacagtttaaaccactgactttaaaaatgtacataaacatggatgccggacatggtgattcaacgattgcacttacagaaacaaatctaagaaaacagtaatgatcttgccagcttctgatgagattataagaaaaaaaaaagaagaaataaatttaaaaaaaaaataaaaaaagaaaatggtaataatccaccaggatgttaataacagcattattcacaagatggaacagaaacaatgattttgtctaacagcagggagttaattaaattatgacaagccagattatagaataatatgcacccattaaatcagagtacttaatgatacggaaaaaattcctattaagtgaaaaaagcattacaaaacagcatatattatgagctctatttttatttttgaaatatatttatgcagagaaatacaaaatgttaacaatattatcttaaaaaaaaaaaataaggctgggcacagtggctcacacctgtaatcccatacttttggaggccaaggtgggtggatcgctttgagcccaggagttcaagaccagcctgggcaacatggcgaaaccccgtctctataaaaaaaattaaaacaattagccaggcatggtagcacacatgtgtagtctcagcaattcgggaggctgcggtgggaggattgcttgagcccaggatattgaggttgcagtgcaatgtgattgtgccactgcactccatcctgggcgacacagcaagaccttttctttaaaaaaaaaaaaaaatcagtttttgctattggtctactcagaatattccagcacttaatttcactattaccatttattctactagtcattctcaactaatgaacatccaaattctctgctaattaagtgcttttaaaagtcacttttgggcgagatgttcaaattaagccctgggtgagagtgccctctggtggtttcccaataatgcttgaacaagaactgtgtagtgagtttttcatgaagctaaatgtatttaaattaaagaagcatcccactttacgaattttaaaatgtctgcaaaacagacaaataagtagatctttcataaaatgttactgatggtggataacaggttcttatccctgggggacgggggaggaacagagggcaggtgatgctggtgatcacggactatgtgcttatttagcaaaattaaaaatcagcaacccatgaaaagcaaaatcccagaaagcacagtgttaatctatacttccagtagaataaagtcaaagttaattctccaaagcactgacacataagtatgtggatgtgggcatcttgggtaaatccttatttagcagagctttgtactcggaagagaagaaaatcttcataatcatattttgatttttcacttctttctacatttataacatagctaagaatttgtagaattttggatataagtcaacctgaaagaaaaccaaacatttttcaagaatacaccatcgacaaagctggtaaatatttctgatttatcaagttcaatcaaacttgtttttttaatctttccaaatgaaatttatattaatggaaaaagtaaaccacttaacagagggtcaccattattaattatttcctttactctctattcctcacacttcactggccacttgaaacttctagagttcctttattaaaataactagatcaaacaatagactttgagaaattatttttcatatcaattttacaaatactgtatcacaaacattctacagtacaaatttaaataaagcaactttctaccttattaaaagattcttcacctcctaaatagaaactgaaggggaagcaatgctattaaggatcatacataagctaatagaggcagcagaattatctattaacattttcctaacactattctagtgaccttaacattttaatcacagagctgcagctgtttgcatgtgttctaaagctagcataatctttaagacagtcaggaaaaaaaaccttcaaaacaaattacataatattctatctagaaaaatttccaggaaagcacattcttgggtgaaagaaaaccacccctttgtcattgtgatgcactaaaaaaaagctttggagcctgatagtttggctcctggctctcccacttgtttgggtaaggttcgagtcactgtaaaatgtaattatactcccttttcaaaggattattttgagaatttaataagaattgatggaaggggcctagcagatagtaaaacctgattaaaatatcactaatttaattatttcctagaagccaactgaaacatcataacatttattttcttggtagaccttatgagtttattctcaaaggcaattaaaaaatctccttcaggaaagccatgcacatttttattaatcatatttatactactaacaatgcttggctgatgattaaaaatacttaaatcacagtagacacacaaaaagagatgtttctcaacttatcatagggttacatcccaataaacctactatcagttgaaaatattgtaaattgaaaatgctagcctgtcttaaatatgctcagaacacttacagtagcctactgtttagcaaaattatctaacacgaagcccgttttataataaagtgttgaatttctgatgtaatttattgatgttctactgaatatgtatggctttggcactatggaaaagtcctaaattggagaccgcacataaatgaaacactaaaatagaaaaagaaaaaagaaaataggtttctctaaatgagaatgtcaaatccagaattactttatataaaagtacacattctaatatatgaaaagatattttatcattattactttactatatattactgaatacaccagactgcattttctcaaatggcaaatgaggcacatttctctttgattcccccaggaacctccgcatcatctgtcttttggaggattcagattcttacgacatctgtgataccgtccatgaggataccaacggtgcttagtagtaaagaacattttgctaagttgttctatcataggtccttcctcaaggtgttcaactttttcttccaatctggttttcagcacttgatcatgtgtttcttcattattatgcacaggatctggccgagggataggttttgtgtgttcatatggaatgtccacagaagggtggtagcatactattgtcctgccatcagaagtcagagcaagctctacgttgcaattatagtcatctggtagaggagaatacgtagatttatgacaaacacaatataaagctccatctattgggtactatgttcactatttgggtgacgggttcagttgaagcccaaacctcagtatatgtaatacatccacgtaacaaacctgcacatgtacgcccgaattttggactggaaataaatgtttcaagatagttctctttgacatcacccattttactgcagctacagccatggtgtttcaagatgcttatcaagtggtatgaaaaaagatgttctgaagagaaactgcttttagaatctgcttctaagcataccaatttctactccttgacggcttctcaccacgaacccgccatcttgtttcaat

SEQ ID NO: 14000 - RNA, 11570 nt, Homo sapiens
  source 1..11570: mol_type = other RNA
gctgggattacaggcatgagccaccgcacccagcccaatgtatatctttataaagctgggaccaaactggcttcttgcagcaataattaaatgttcaaatatgctcaacagaactttccctctagataatcatcatatctctaaatgtaatcacagttgtttgttttccaaactattacataaagagaacaatctcaaacttattgcattagcctttacacaagttatgttctttactaagtcactgaacacactgtacagttcagttgatatgctttttctaccaagactttttcaaataaaaagatatagtaggttgatttacattctagggcaagctccttaatttaggtaattattccggaatgttctcttaccactgctgctatccatccaattggattcctacaaagcttcaaaccacattaattaacaaagtaatttattccacactttactgttgtttagagttagctgtttgttggcaatgaagtggaaaaaagagaatcttccttcatattactatcatattcaaatagcatataaactaattgccatattagtaatatctatatattaatggtacatcaaaccaattgcaagaaaaggtaatttattagctttctttgttctatgggttgatcttcctggatatttcaaattgttgtgtgttggtaactggtaattgaagtactttctttgccacacagtctcccaacatttctaagaatctttgatgctgattattattaagacaattattgtctatatataagattattgtcttaattgcattttttagttttagcaatctaaagttgcttaaagatgtctaaaaagcattaacgtttatttgtgaaataatgaatatctgtgctttcagttttttaattacttaggtttttctttcaaagagatcttctggttttggatttatctctttatgttctgtatttaaatgttgatttagttttgattattttattgcttcatttgccagaacttctcagcaaataacatgttatggttttcccatgtcttcatttatggctaaaaaactgaactcagtatatgaagaattatatttatgagtaaaactagaacaatctattggttttcatttattcagaatcgcttttattgtcaccattaggtttactaatactgttgcattcagaaaaggtaagtcttttcttgataaaaaaagccagtgaagttattttgccatccataacatggtgttaaagataaatgaaacaaattaccccaaaccttcacatcgattgcattccctgcctgaaactttctctcctttctctttaaacagatctaatcttaacactggtcccccataaaaatatttccagtgcatatatctgacaaaagatttatccaaaatatttaaagaaatattataacttcaatcataagaagaaaaaataatgagtaaatagatgttccatatcacatattatcagggaaatgcaaattaaaataaatgtgatgtggatgagctgtctgagcagagaaaaacacaaaacaagtgagacaccactacacaccttttagaatggccaaaattcagaacactaacaccaagtgctgacagggatgttgagcaataggaacccttattcactgctggtgggaatgcaaaatggtacagcctctctgtaggacagtttggtggttttttacaaaacgaaacattctcttagcattcaatccaacaattgtgctctttggtatttacccaaaggagttgaaagcttaaatggacacaaaaacctacacatggatatctatagcaattttattcataattgccaaaacttggaagcaatcaaccaagatgtccttcagcaggtgaatggataaactgttgtacacccagacaatggagtattactcgatgctaaaaagaaatgagctatcaaactgtgaaaagacatagaggaaacaaatgcatattatccagtgaaagaaaccaatgtgaaaaggctatatatactttatgattccaactatatggcgttctgaaaaaggaaaaacttacggagacagtgaaaagaccagtggtagccgggggtcagtggggaggacacgacgaagaggcagagccaagggtttttaggacagtgtagactctgcatgactataaagatggatacatgtcattgtacctttgttcaaacccatagattgtacagcaccaagagtgaaccctaatggaaacaataggctttgggtgataatgatgtgtcagtgtaggtttatcaattgtaaccaatgtgccactctgctgggggatggtgatgagggaggcatgggggaggggagcactgaggatatataagttatttctgtaccctcctctcaattttgctcagaacctaaaactacttttaaaaactaaagttttttttttttttcaggagatgaggatctcactatgttgcccaggctgcagtgcagtggctattcacaggtgtgatcccactactgatcagcacaggagttttgacctgctccacttctgacgctccttaggcaactctgggtcccagtgacccaggaggtcactacatttatgctgaacttagtgcaaacacctgattgacatagctcactacaacccagaacttctggactcaagtgatcctcctgtcttagcctcctgagtagctaggtctacaggcatgtgccactgtgcctggcaaaaagtcttttttaagtgctaagaaaaaaaaaagagcaaatgatttgaacagatatttcaccaaagatatgagtgcccaacaagtacctgaatcaaaacttaatgttattgatcatcagagaaatgcaaattaaaaccatcaaattattactatatatccattagaatggctaaaactaaaaatattatcaaatgagggcaagaatatagcaattggaactttcattcatggtggtgagaatataaaatggtacaaccactttgcaaaaagcgttttggcagttttttttttttttttgagacggaatctcgttttatcacccagactggagtgcagtggtgtgatcttggcccactgcaacctctgcctcctgggttcaagggattctcctgcctcagcctcctgagtagctaggattacagatgcctgccaccacacccagctaatttttgcatttttagtagagacggggtttcaccatgttagctaggctggtctcaaactcctgacctcaagtgatccgcccacctccgcctcctaaagtgctgggattacaggtgtgaactaccacgcccagccccccagctcattcttagctaactagtgtgtgtgaaaaagagacagtgttaaaatatatatggtttaaactgataaggaaatgatcagttattgagcttatccatgattgctaattcaggtagagatggcttataagtaagtgttcggggctgcttacgggaagaaaaaatgaaagttagggatttcctttggatgctgggaaacaaaactccaactgggttctgacaaacataccatgtgcattgtcctgtggagacatgacaatgtaaacccataaacaaatcgattacgttttggtgacaactattgtgaagagaatggccatagtatttgctgcttctccttttaataggtagcatctctcctcttactcccttgaatctgagatagccttatgaagtgatattgtgccagttctgagactaggcctcaagaagcctcgaagcttccaatcttgcacttttttgtttgttttgatacaggtgcttgttctgttgcccagcctagagtgcagtggcacaatcatggctcactacagcctcaatctcatgggctcaagcaatcctcccatctcagcctcccaaatagctgggactacaggcatgcagcaccaccccaccctccccacccccagctaattttttaaaatttttttgtagaagaccaggcgtggtggctcacacctgtaatcccagcactttgggaggctgaggcaggcagatcacctgaggtggggaattcaagaccagcctgaccaacacggagaaacccatctctactaaaaatacaaaattagctgggcgtggtggctcatgcctgtaatctcagctactcaggagactgaggcaggagaatcgcttgaacccaagaggcaaaggttctggtgggctgagattgcgccattgcactccagcctgggcaacaagggcgaaactccatctcaaaaaatttttttttttacagatgggctctcactatgttgcccaggctggtcttgaactcctgggctcaagaaatcccccaaccttggcctcccaaagtgctgggattacaggtgtgagtcatcatgcccagccccaatctcatactcttgaaatcctaaagccatgtgaagaatccaggcctagcttgctggatgatgagagacacagtccccctaatgccccaggtgacagtcactcaataccagacatatgagtgacaccatctaggactagccagcctcaacaacccaactagtgacctcagctgcatgggcaagtccagccaagataagctgagctggatccagactataagaattacctggaagaacgcaaactaatgaaagattgttgttttaagccaatgagctttggggtgatttgttaattggcaatagataactgatattcaaggattcatccaaagttcccttaaaagatagaacccattaagtcattttaaacacttataagcaagttattaaatccttaaaagaaactgaaagtttctaaggtatactgggttggaaaaaggaaaagaaaaagaaactaaaagtgaaggctgaaactgacaagtaaggagttatttctccctgcaaatgtaatcagaaaataaggtggagtgtctctgaatgcataactggaacaaggaaacaatctaatggttttagtagtaaatatatgatttcaggggcacatccagtggaatgatggagtcagtgcacaacaacttgtaagacccagtcatggaaactggcaaacattacaagttagaaccagttgttaaatcttcattagtacatcactggacacatctattgctaaaggcacatttcatcagtatgtatatgcataaatatacatataagatgtccttaatgtttaaaaaagacattggttggttctgccacaatctgtgatcttgggcaagtcaattagtgtctttggatctgtttccaaatcagtccccaaaaatcatctttaagatgtctttcagctttacgattctatcttctatgctcttatggtaattacacctggatgcagcaattgaaaagtccaatgggatcaatccaaattgccacacttaaccatgttactgactacatatattactcatcaagacaattattcaagtaagtggcataatagtaatccaatgtactttgcattatgagtgaagaagagactaattttgactagaggggaaagaagggatggtcatagcaagatactttgtcaatcaggaatgagggctatctttgaacccacagtggcttgaactctataggtgcttaataaaatttgccgaaaagattacatgcttagagacaacattataaagaaaagacattcttggccgggcgtggtggctcatgcctgtaatcccagcacttcaggaggcgaaagcaggtggatcacctgaggtcaggagtttgagaccagcctgaccaacatggagaaaccccatctctactaaatacaaaaaattagccggacatggtgttgcatgcctatagtcccagctacttgggaagctgaggcaggagaatcgcttgaacccgggaggtggaggttgcagtgagctgagaatgtgccactacactccagccaaggcaacaagagcaagactctgtcccaaaaaaaaaaaaaaaaaaaaaagagacattcttgctgaattgaagactcagaagaggctgggcacagtggctcacccttgtaatcccagtattttggggggccaaggtgggcagatcacctgaggtcaggagttcaagaccagcctggccaacgtggtgaaaccccatctctactgaaaatacaaaaaatcagccaggcatgctggtgcacgctcataatcccagctactcgggaggctgaggcaggagaattgcttgagcctatgaggcggaggttgcagtgggctgagatcatgccactggccactgtactgcactccagcctgggtgacaaaagtgaaactccatctcaaaaaaaaaaaaaaaaaaaagactcagaagtaatcataaggttctacttgctattctcacatgtaattgtgagactctgcctccatttctccatctaaaaacaggagctcatttacaagcaacatgacaagaattcaagcagtcatggctgtgaagcatttctgcagaaggatatgctatgtaagtatgaggttgttactaaatcaaaatgaatgcctttgtgcaaaactagaaagcacattacatattgttcctgagtattccttcccagtgcattcaaaatattctcacattcacaaggttaaacagcacattaaaaaatagtaggaggctgatggctgagctcaattgggagtatctttctttggtgttagaatgtttgaaaattattttgggaagactatgagcaagttattttgaacttctggggaaaaaaaaaaatctgaagaagcattccctttgcctaaaagcaaaggagacatttatttatgcctttagcaaataaaatagtttgcttactaccagtgtttgtgggctgatattcaactcatcttctggaaattttaaaaatacacattgaaactgaaaaagtattctttgagtaagggtttacctgaagtgcccagaaccatccaaaatgatggcacattatatctttttttcttaaaaatttttggaatctaattgaagatgcctcttagaatatgtggaaaccacacgtgctatcttgcatatcactatcatttcagttctaatgttattaggtgtttagctacaggcaagtagaattagggcatgatgtgacagactgtaatgagttgctgagaaactacatactctatccccaggaaaacacatattctcaaaattctacacaatttcaggaatttcatagatgcccctaccccaaatcccattcatgaaatccttagcttaaaatcctgtgcactagagcaatgtattttataaaaccatattcagatgcctgtgaagcaatgaatgtgctaggcaatgttaggcggtagaaacagtgatacacgtagtcagacagggtacctagaagtcatggagcttataggctagtaggggatatggacatttaccaaataatcacacaaaaagatgcctaattacaaactctgattaagtgctatggagagatatacagtgttgcacgtaacaacagaatctaaagaagttacattttagggggcatataaacaatgttgtgcaggggaggtagaagaaacacattatggtaaagggctgcaaaggaaataagcccataataaggcctcttataggtttaagctaggacctgaaacttgtatactttatatgctttgaaatgagacatacattaaagtggctgatcaaattaaaacattttccagtctttgcctactaaattgataaagattttttaaaattttaatagaactaaagagaaaatatttctatatactgatgttaggagtatgcagtttaggccaggcatggaggctcacacctataatcccacccagcactttgggaggccaaggtgtgtggacacttgaggtcaggagttcgagaccagcctgaccaacatggtgaaaccctgtctctactaaaaatgcaaaattacctgagtatggtggtgcacacttgtaatcccaactacttaaggaggctgaggcaggagaatcacttgaacccgggaggtggaggctgcagtgagccaagatcgcgccattgcattccagcttgggcagagcaaacctccatctccaaaacccaaaaagtatacagtttaaaccactgactttaaaaatgtacataaacatggatgccggacatggtgattcaacgattgcacttacagaaacaaatctaagaaaacagtaatgatcttgccagcttctgatgagattataagaaaaaaaaaagaagaaataaatttaaaaaaaaaataaaaaaagaaaatggtaataatccaccaggatgttaataacagcattattcacaagatggaacagaaacaatgattttgtctaacagcagggagttaattaaattatgacaagccagattatagaataatatgcacccattaaatcagagtacttaatgatacggaaaaaattcctattaagtgaaaaaagcattacaaaacagcatatattatgagctctatttttatttttgaaatatatttatgcagagaaatacaaaatgttaacaatattatcttaaaaaaaaaaaataaggctgggcacagtggctcacacctgtaatcccatacttttggaggccaaggtgggtggatcgctttgagcccaggagttcaagaccagcctgggcaacatggcgaaaccccgtctctataaaaaaaattaaaacaattagccaggcatggtagcacacatgtgtagtctcagcaattcgggaggctgcggtgggaggattgcttgagcccaggatattgaggttgcagtgcaatgtgattgtgccactgcactccatcctgggcgacacagcaagaccttttctttaaaaaaaaaaaaaaatcagtttttgctattggtctactcagaatattccagcacttaatttcactattaccatttattctactagtcattctcaactaatgaacatccaaattctctgctaattaagtgcttttaaaagtcacttttgggcgagatgttcaaattaagccctgggtgagagtgccctctggtggtttcccaataatgcttgaacaagaactgtgtagtgagtttttcatgaagctaaatgtatttaaattaaagaagcatcccactttacgaattttaaaatgtctgcaaaacagacaaataagtagatctttcataaaatgttactgatggtggataacaggttcttatccctgggggacgggggaggaacagagggcaggtgatgctggtgatcacggactatgtgcttatttagcaaaattaaaaatcagcaacccatgaaaagcaaaatcccagaaagcacagtgttaatctatacttccagtagaataaagtcaaagttaattctccaaagcactgacacataagtatgtggatgtgggcatcttgggtaaatccttatttagcagagctttgtactcggaagagaagaaaatcttcataatcatattttgatttttcacttctttctacatttataacatagctaagaatttgtagaattttggatataagtcaacctgaaagaaaaccaaacatttttcaagaatacaccatcgacaaagctggtaaatatttctgatttatcaagttcaatcaaacttgtttttttaatctttccaaatgaaatttatattaatggaaaaagtaaaccacttaacagagggtcaccattattaattatttcctttactctctattcctcacacttcactggccacttgaaacttctagagttcctttattaaaataactagatcaaacaatagactttgagaaattatttttcatatcaattttacaaatactgtatcacaaacattctacagtacaaatttaaataaagcaactttctaccttattaaaagattcttcacctcctaaatagaaactgaaggggaagcaatgctattaaggatcatacataagctaatagaggcagcagaattatctattaacattttcctaacactattctagtgaccttaacattttaatcacagagctgcagctgtttgcatgtgttctaaagctagcataatctttaagacagtcaggaaaaaaaaccttcaaaacaaattacataatattctatctagaaaaatttccaggaaagcacattcttgggtgaaagaaaaccacccctttgtcattgtgatgcactaaaaaaaagctttggagcctgatagtttggctcctggctctcccacttgtttgggtaaggttcgagtcactgtaaaatgtaattatactcccttttcaaaggattattttgagaatttaataagaattgatggaaggggcctagcagatagtaaaacctgattaaaatatcactaatttaattatttcctagaagccaactgaaacatcataacatttattttcttggtagaccttatgagtttattctcaaaggcaattaaaaaatctccttcaggaaagccatgcacatttttattaatcatatttatactactaacaatgcttggctgatgattaaaaatacttaaatcacagtagacacacaaaaagagatgtttctcaacttatcatagggttacatcccaataaacctactatcagttgaaaatattgtaaattgaaaatgctagcctgtcttaaatatgctcagaacacttacagtagcctactgtttagcaaaattatctaacacgaagcccgttttataataaagtgttgaatttctgatgtaatttattgatgttctactgaatatgtatggctttggcactatggaaaagtcctaaattggagaccgcacataaatgaaacactaaaatagaaaaagaaaaaagaaaataggtttctctaaatgagaatgtcaaatccagaattactttatataaaagtacacattctaatatatgaaaagatattttatcattattactttactatatattactgaatacaccagactgcattttctcaaatggcaaatgaggcacatttctctttgattcccccaggaacctccgcatcatctgtcttttggaggattcagattcttacgacatctgtgataccgtccatgaggataccaacggtgcttagtagtaaagaacattttgctaagttgttctatcataggtccttcctcaaggtgttcaactttttcttccaatctggttttcagcacttgatcatgtgtttcttcattattatgcacaggatctggccgagggataggttttgtgtgttcatatggaatgtccacagaagggtggtagcatactattgtcctgccatcagaagtcagagcaagctctacgttgcaattatagtcatctggtagaggagaatacgtagatttatgacaaacacaatataaagctccatctgcacatgtacgcccgaattttggactggaaataaatgtttcaagatagttctctttgacatcacccattttactgcagctacagccatggtgtttcaagatgcttatcaagtggtatgaaaaaagatgttctgaagagaaactgcttttagaatctgcttctaagcataccaatttctactcctgcttgacggcttctcaccacgaacccgccatcttgtttcaat

SEQ ID NO: 14001 - RNA, 11567 nt, Homo sapiens
  source 1..11567: mol_type = other RNA
gctgggattacaggcatgagccaccgcacccagcccaatgtatatctttataaagctgggaccaaactggcttcttgcagcaataattaaatgttcaaatatgctcaacagaactttccctctagataatcatcatatctctaaatgtaatcacagttgtttgttttccaaactattacataaagagaacaatctcaaacttattgcattagcctttacacaagttatgttctttactaagtcactgaacacactgtacagttcagttgatatgctttttctaccaagactttttcaaataaaaagatatagtaggttgatttacattctagggcaagctccttaatttaggtaattattccggaatgttctcttaccactgctgctatccatccaattggattcctacaaagcttcaaaccacattaattaacaaagtaatttattccacactttactgttgtttagagttagctgtttgttggcaatgaagtggaaaaaagagaatcttccttcatattactatcatattcaaatagcatataaactaattgccatattagtaatatctatatattaatggtacatcaaaccaattgcaagaaaaggtaatttattagctttctttgttctatgggttgatcttcctggatatttcaaattgttgtgtgttggtaactggtaattgaagtactttctttgccacacagtctcccaacatttctaagaatctttgatgctgattattattaagacaattattgtctatatataagattattgtcttaattgcattttttagttttagcaatctaaagttgcttaaagatgtctaaaaagcattaacgtttatttgtgaaataatgaatatctgtgctttcagttttttaattacttaggtttttctttcaaagagatcttctggttttggatttatctctttatgttctgtatttaaatgttgatttagttttgattattttattgcttcatttgccagaacttctcagcaaataacatgttatggttttcccatgtcttcatttatggctaaaaaactgaactcagtatatgaagaattatatttatgagtaaaactagaacaatctattggttttcatttattcagaatcgcttttattgtcaccattaggtttactaatactgttgcattcagaaaaggtaagtcttttcttgataaaaaaagccagtgaagttattttgccatccataacatggtgttaaagataaatgaaacaaattaccccaaaccttcacatcgattgcattccctgcctgaaactttctctcctttctctttaaacagatctaatcttaacactggtcccccataaaaatatttccagtgcatatatctgacaaaagatttatccaaaatatttaaagaaatattataacttcaatcataagaagaaaaaataatgagtaaatagatgttccatatcacatattatcagggaaatgcaaattaaaataaatgtgatgtggatgagctgtctgagcagagaaaaacacaaaacaagtgagacaccactacacaccttttagaatggccaaaattcagaacactaacaccaagtgctgacagggatgttgagcaataggaacccttattcactgctggtgggaatgcaaaatggtacagcctctctgtaggacagtttggtggttttttacaaaacgaaacattctcttagcattcaatccaacaattgtgctctttggtatttacccaaaggagttgaaagcttaaatggacacaaaaacctacacatggatatctatagcaattttattcataattgccaaaacttggaagcaatcaaccaagatgtccttcagcaggtgaatggataaactgttgtacacccagacaatggagtattactcgatgctaaaaagaaatgagctatcaaactgtgaaaagacatagaggaaacaaatgcatattatccagtgaaagaaaccaatgtgaaaaggctatatatactttatgattccaactatatggcgttctgaaaaaggaaaaacttacggagacagtgaaaagaccagtggtagccgggggtcagtggggaggacacgacgaagaggcagagccaagggtttttaggacagtgtagactctgcatgactataaagatggatacatgtcattgtacctttgttcaaacccatagattgtacagcaccaagagtgaaccctaatggaaacaataggctttgggtgataatgatgtgtcagtgtaggtttatcaattgtaaccaatgtgccactctgctgggggatggtgatgagggaggcatgggggaggggagcactgaggatatataagttatttctgtaccctcctctcaattttgctcagaacctaaaactacttttaaaaactaaagttttttttttttttcaggagatgaggatctcactatgttgcccaggctgcagtgcagtggctattcacaggtgtgatcccactactgatcagcacaggagttttgacctgctccacttctgacgctccttaggcaactctgggtcccagtgacccaggaggtcactacatttatgctgaacttagtgcaaacacctgattgacatagctcactacaacccagaacttctggactcaagtgatcctcctgtcttagcctcctgagtagctaggtctacaggcatgtgccactgtgcctggcaaaaagtcttttttaagtgctaagaaaaaaaaaagagcaaatgatttgaacagatatttcaccaaagatatgagtgcccaacaagtacctgaatcaaaacttaatgttattgatcatcagagaaatgcaaattaaaaccatcaaattattactatatatccattagaatggctaaaactaaaaatattatcaaatgagggcaagaatatagcaattggaactttcattcatggtggtgagaatataaaatggtacaaccactttgcaaaaagcgttttggcagttttttttttttttttgagacggaatctcgttttatcacccagactggagtgcagtggtgtgatcttggcccactgcaacctctgcctcctgggttcaagggattctcctgcctcagcctcctgagtagctaggattacagatgcctgccaccacacccagctaatttttgcatttttagtagagacggggtttcaccatgttagctaggctggtctcaaactcctgacctcaagtgatccgcccacctccgcctcctaaagtgctgggattacaggtgtgaactaccacgcccagccccccagctcattcttagctaactagtgtgtgtgaaaaagagacagtgttaaaatatatatggtttaaactgataaggaaatgatcagttattgagcttatccatgattgctaattcaggtagagatggcttataagtaagtgttcggggctgcttacgggaagaaaaaatgaaagttagggatttcctttggatgctgggaaacaaaactccaactgggttctgacaaacataccatgtgcattgtcctgtggagacatgacaatgtaaacccataaacaaatcgattacgttttggtgacaactattgtgaagagaatggccatagtatttgctgcttctccttttaataggtagcatctctcctcttactcccttgaatctgagatagccttatgaagtgatattgtgccagttctgagactaggcctcaagaagcctcgaagcttccaatcttgcacttttttgtttgttttgatacaggtgcttgttctgttgcccagcctagagtgcagtggcacaatcatggctcactacagcctcaatctcatgggctcaagcaatcctcccatctcagcctcccaaatagctgggactacaggcatgcagcaccaccccaccctccccacccccagctaattttttaaaatttttttgtagaagaccaggcgtggtggctcacacctgtaatcccagcactttgggaggctgaggcaggcagatcacctgaggtggggaattcaagaccagcctgaccaacacggagaaacccatctctactaaaaatacaaaattagctgggcgtggtggctcatgcctgtaatctcagctactcaggagactgaggcaggagaatcgcttgaacccaagaggcaaaggttctggtgggctgagattgcgccattgcactccagcctgggcaacaagggcgaaactccatctcaaaaaatttttttttttacagatgggctctcactatgttgcccaggctggtcttgaactcctgggctcaagaaatcccccaaccttggcctcccaaagtgctgggattacaggtgtgagtcatcatgcccagccccaatctcatactcttgaaatcctaaagccatgtgaagaatccaggcctagcttgctggatgatgagagacacagtccccctaatgccccaggtgacagtcactcaataccagacatatgagtgacaccatctaggactagccagcctcaacaacccaactagtgacctcagctgcatgggcaagtccagccaagataagctgagctggatccagactataagaattacctggaagaacgcaaactaatgaaagattgttgttttaagccaatgagctttggggtgatttgttaattggcaatagataactgatattcaaggattcatccaaagttcccttaaaagatagaacccattaagtcattttaaacacttataagcaagttattaaatccttaaaagaaactgaaagtttctaaggtatactgggttggaaaaaggaaaagaaaaagaaactaaaagtgaaggctgaaactgacaagtaaggagttatttctccctgcaaatgtaatcagaaaataaggtggagtgtctctgaatgcataactggaacaaggaaacaatctaatggttttagtagtaaatatatgatttcaggggcacatccagtggaatgatggagtcagtgcacaacaacttgtaagacccagtcatggaaactggcaaacattacaagttagaaccagttgttaaatcttcattagtacatcactggacacatctattgctaaaggcacatttcatcagtatgtatatgcataaatatacatataagatgtccttaatgtttaaaaaagacattggttggttctgccacaatctgtgatcttgggcaagtcaattagtgtctttggatctgtttccaaatcagtccccaaaaatcatctttaagatgtctttcagctttacgattctatcttctatgctcttatggtaattacacctggatgcagcaattgaaaagtccaatgggatcaatccaaattgccacacttaaccatgttactgactacatatattactcatcaagacaattattcaagtaagtggcataatagtaatccaatgtactttgcattatgagtgaagaagagactaattttgactagaggggaaagaagggatggtcatagcaagatactttgtcaatcaggaatgagggctatctttgaacccacagtggcttgaactctataggtgcttaataaaatttgccgaaaagattacatgcttagagacaacattataaagaaaagacattcttggccgggcgtggtggctcatgcctgtaatcccagcacttcaggaggcgaaagcaggtggatcacctgaggtcaggagtttgagaccagcctgaccaacatggagaaaccccatctctactaaatacaaaaaattagccggacatggtgttgcatgcctatagtcccagctacttgggaagctgaggcaggagaatcgcttgaacccgggaggtggaggttgcagtgagctgagaatgtgccactacactccagccaaggcaacaagagcaagactctgtcccaaaaaaaaaaaaaaaaaaaaaagagacattcttgctgaattgaagactcagaagaggctgggcacagtggctcacccttgtaatcccagtattttggggggccaaggtgggcagatcacctgaggtcaggagttcaagaccagcctggccaacgtggtgaaaccccatctctactgaaaatacaaaaaatcagccaggcatgctggtgcacgctcataatcccagctactcgggaggctgaggcaggagaattgcttgagcctatgaggcggaggttgcagtgggctgagatcatgccactggccactgtactgcactccagcctgggtgacaaaagtgaaactccatctcaaaaaaaaaaaaaaaaaaaagactcagaagtaatcataaggttctacttgctattctcacatgtaattgtgagactctgcctccatttctccatctaaaaacaggagctcatttacaagcaacatgacaagaattcaagcagtcatggctgtgaagcatttctgcagaaggatatgctatgtaagtatgaggttgttactaaatcaaaatgaatgcctttgtgcaaaactagaaagcacattacatattgttcctgagtattccttcccagtgcattcaaaatattctcacattcacaaggttaaacagcacattaaaaaatagtaggaggctgatggctgagctcaattgggagtatctttctttggtgttagaatgtttgaaaattattttgggaagactatgagcaagttattttgaacttctggggaaaaaaaaaaatctgaagaagcattccctttgcctaaaagcaaaggagacatttatttatgcctttagcaaataaaatagtttgcttactaccagtgtttgtgggctgatattcaactcatcttctggaaattttaaaaatacacattgaaactgaaaaagtattctttgagtaagggtttacctgaagtgcccagaaccatccaaaatgatggcacattatatctttttttcttaaaaatttttggaatctaattgaagatgcctcttagaatatgtggaaaccacacgtgctatcttgcatatcactatcatttcagttctaatgttattaggtgtttagctacaggcaagtagaattagggcatgatgtgacagactgtaatgagttgctgagaaactacatactctatccccaggaaaacacatattctcaaaattctacacaatttcaggaatttcatagatgcccctaccccaaatcccattcatgaaatccttagcttaaaatcctgtgcactagagcaatgtattttataaaaccatattcagatgcctgtgaagcaatgaatgtgctaggcaatgttaggcggtagaaacagtgatacacgtagtcagacagggtacctagaagtcatggagcttataggctagtaggggatatggacatttaccaaataatcacacaaaaagatgcctaattacaaactctgattaagtgctatggagagatatacagtgttgcacgtaacaacagaatctaaagaagttacattttagggggcatataaacaatgttgtgcaggggaggtagaagaaacacattatggtaaagggctgcaaaggaaataagcccataataaggcctcttataggtttaagctaggacctgaaacttgtatactttatatgctttgaaatgagacatacattaaagtggctgatcaaattaaaacattttccagtctttgcctactaaattgataaagattttttaaaattttaatagaactaaagagaaaatatttctatatactgatgttaggagtatgcagtttaggccaggcatggaggctcacacctataatcccacccagcactttgggaggccaaggtgtgtggacacttgaggtcaggagttcgagaccagcctgaccaacatggtgaaaccctgtctctactaaaaatgcaaaattacctgagtatggtggtgcacacttgtaatcccaactacttaaggaggctgaggcaggagaatcacttgaacccgggaggtggaggctgcagtgagccaagatcgcgccattgcattccagcttgggcagagcaaacctccatctccaaaacccaaaaagtatacagtttaaaccactgactttaaaaatgtacataaacatggatgccggacatggtgattcaacgattgcacttacagaaacaaatctaagaaaacagtaatgatcttgccagcttctgatgagattataagaaaaaaaaaagaagaaataaatttaaaaaaaaaataaaaaaagaaaatggtaataatccaccaggatgttaataacagcattattcacaagatggaacagaaacaatgattttgtctaacagcagggagttaattaaattatgacaagccagattatagaataatatgcacccattaaatcagagtacttaatgatacggaaaaaattcctattaagtgaaaaaagcattacaaaacagcatatattatgagctctatttttatttttgaaatatatttatgcagagaaatacaaaatgttaacaatattatcttaaaaaaaaaaaataaggctgggcacagtggctcacacctgtaatcccatacttttggaggccaaggtgggtggatcgctttgagcccaggagttcaagaccagcctgggcaacatggcgaaaccccgtctctataaaaaaaattaaaacaattagccaggcatggtagcacacatgtgtagtctcagcaattcgggaggctgcggtgggaggattgcttgagcccaggatattgaggttgcagtgcaatgtgattgtgccactgcactccatcctgggcgacacagcaagaccttttctttaaaaaaaaaaaaaaatcagtttttgctattggtctactcagaatattccagcacttaatttcactattaccatttattctactagtcattctcaactaatgaacatccaaattctctgctaattaagtgcttttaaaagtcacttttgggcgagatgttcaaattaagccctgggtgagagtgccctctggtggtttcccaataatgcttgaacaagaactgtgtagtgagtttttcatgaagctaaatgtatttaaattaaagaagcatcccactttacgaattttaaaatgtctgcaaaacagacaaataagtagatctttcataaaatgttactgatggtggataacaggttcttatccctgggggacgggggaggaacagagggcaggtgatgctggtgatcacggactatgtgcttatttagcaaaattaaaaatcagcaacccatgaaaagcaaaatcccagaaagcacagtgttaatctatacttccagtagaataaagtcaaagttaattctccaaagcactgacacataagtatgtggatgtgggcatcttgggtaaatccttatttagcagagctttgtactcggaagagaagaaaatcttcataatcatattttgatttttcacttctttctacatttataacatagctaagaatttgtagaattttggatataagtcaacctgaaagaaaaccaaacatttttcaagaatacaccatcgacaaagctggtaaatatttctgatttatcaagttcaatcaaacttgtttttttaatctttccaaatgaaatttatattaatggaaaaagtaaaccacttaacagagggtcaccattattaattatttcctttactctctattcctcacacttcactggccacttgaaacttctagagttcctttattaaaataactagatcaaacaatagactttgagaaattatttttcatatcaattttacaaatactgtatcacaaacattctacagtacaaatttaaataaagcaactttctaccttattaaaagattcttcacctcctaaatagaaactgaaggggaagcaatgctattaaggatcatacataagctaatagaggcagcagaattatctattaacattttcctaacactattctagtgaccttaacattttaatcacagagctgcagctgtttgcatgtgttctaaagctagcataatctttaagacagtcaggaaaaaaaaccttcaaaacaaattacataatattctatctagaaaaatttccaggaaagcacattcttgggtgaaagaaaaccacccctttgtcattgtgatgcactaaaaaaaagctttggagcctgatagtttggctcctggctctcccacttgtttgggtaaggttcgagtcactgtaaaatgtaattatactcccttttcaaaggattattttgagaatttaataagaattgatggaaggggcctagcagatagtaaaacctgattaaaatatcactaatttaattatttcctagaagccaactgaaacatcataacatttattttcttggtagaccttatgagtttattctcaaaggcaattaaaaaatctccttcaggaaagccatgcacatttttattaatcatatttatactactaacaatgcttggctgatgattaaaaatacttaaatcacagtagacacacaaaaagagatgtttctcaacttatcatagggttacatcccaataaacctactatcagttgaaaatattgtaaattgaaaatgctagcctgtcttaaatatgctcagaacacttacagtagcctactgtttagcaaaattatctaacacgaagcccgttttataataaagtgttgaatttctgatgtaatttattgatgttctactgaatatgtatggctttggcactatggaaaagtcctaaattggagaccgcacataaatgaaacactaaaatagaaaaagaaaaaagaaaataggtttctctaaatgagaatgtcaaatccagaattactttatataaaagtacacattctaatatatgaaaagatattttatcattattactttactatatattactgaatacaccagactgcattttctcaaatggcaaatgaggcacatttctctttgattcccccaggaacctccgcatcatctgtcttttggaggattcagattcttacgacatctgtgataccgtccatgaggataccaacggtgcttagtagtaaagaacattttgctaagttgttctatcataggtccttcctcaaggtgttcaactttttcttccaatctggttttcagcacttgatcatgtgtttcttcattattatgcacaggatctggccgagggataggttttgtgtgttcatatggaatgtccacagaagggtggtagcatactattgtcctgccatcagaagtcagagcaagctctacgttgcaattatagtcatctggtagaggagaatacgtagatttatgacaaacacaatataaagctccatctgcacatgtacgcccgaattttggactggaaataaatgtttcaagatagttctctttgacatcacccattttactgcagctacagccatggtgtttcaagatgcttatcaagtggtatgaaaaaagatgttctgaagagaaactgcttttagaatctgcttctaagcataccaatttctactccttgacggcttctcaccacgaacccgccatcttgtttcaat

SEQ ID NO: 14002 - RNA, 11550 nt, Homo sapiens
  source 1..11550: mol_type = other RNA
gctgggattacaggcatgagccaccgcacccagcccaatgtatatctttataaagctgggaccaaactggcttcttgcagcaataattaaatgttcaaatatgctcaacagaactttccctctagataatcatcatatctctaaatgtaatcacagttgtttgttttccaaactattacataaagagaacaatctcaaacttattgcattagcctttacacaagttatgttctttactaagtcactgaacacactgtacagttcagttgatatgctttttctaccaagactttttcaaataaaaagatatagtaggttgatttacattctagggcaagctccttaatttaggtaattattccggaatgttctcttaccactgctgctatccatccaattggattcctacaaagcttcaaaccacattaattaacaaagtaatttattccacactttactgttgtttagagttagctgtttgttggcaatgaagtggaaaaaagagaatcttccttcatattactatcatattcaaatagcatataaactaattgccatattagtaatatctatatattaatggtacatcaaaccaattgcaagaaaaggtaatttattagctttctttgttctatgggttgatcttcctggatatttcaaattgttgtgtgttggtaactggtaattgaagtactttctttgccacacagtctcccaacatttctaagaatctttgatgctgattattattaagacaattattgtctatatataagattattgtcttaattgcattttttagttttagcaatctaaagttgcttaaagatgtctaaaaagcattaacgtttatttgtgaaataatgaatatctgtgctttcagttttttaattacttaggtttttctttcaaagagatcttctggttttggatttatctctttatgttctgtatttaaatgttgatttagttttgattattttattgcttcatttgccagaacttctcagcaaataacatgttatggttttcccatgtcttcatttatggctaaaaaactgaactcagtatatgaagaattatatttatgagtaaaactagaacaatctattggttttcatttattcagaatcgcttttattgtcaccattaggtttactaatactgttgcattcagaaaaggtaagtcttttcttgataaaaaaagccagtgaagttattttgccatccataacatggtgttaaagataaatgaaacaaattaccccaaaccttcacatcgattgcattccctgcctgaaactttctctcctttctctttaaacagatctaatcttaacactggtcccccataaaaatatttccagtgcatatatctgacaaaagatttatccaaaatatttaaagaaatattataacttcaatcataagaagaaaaaataatgagtaaatagatgttccatatcacatattatcagggaaatgcaaattaaaataaatgtgatgtggatgagctgtctgagcagagaaaaacacaaaacaagtgagacaccactacacaccttttagaatggccaaaattcagaacactaacaccaagtgctgacagggatgttgagcaataggaacccttattcactgctggtgggaatgcaaaatggtacagcctctctgtaggacagtttggtggttttttacaaaacgaaacattctcttagcattcaatccaacaattgtgctctttggtatttacccaaaggagttgaaagcttaaatggacacaaaaacctacacatggatatctatagcaattttattcataattgccaaaacttggaagcaatcaaccaagatgtccttcagcaggtgaatggataaactgttgtacacccagacaatggagtattactcgatgctaaaaagaaatgagctatcaaactgtgaaaagacatagaggaaacaaatgcatattatccagtgaaagaaaccaatgtgaaaaggctatatatactttatgattccaactatatggcgttctgaaaaaggaaaaacttacggagacagtgaaaagaccagtggtagccgggggtcagtggggaggacacgacgaagaggcagagccaagggtttttaggacagtgtagactctgcatgactataaagatggatacatgtcattgtacctttgttcaaacccatagattgtacagcaccaagagtgaaccctaatggaaacaataggctttgggtgataatgatgtgtcagtgtaggtttatcaattgtaaccaatgtgccactctgctgggggatggtgatgagggaggcatgggggaggggagcactgaggatatataagttatttctgtaccctcctctcaattttgctcagaacctaaaactacttttaaaaactaaagttttttttttttttcaggagatgaggatctcactatgttgcccaggctgcagtgcagtggctattcacaggtgtgatcccactactgatcagcacaggagttttgacctgctccacttctgacgctccttaggcaactctgggtcccagtgacccaggaggtcactacatttatgctgaacttagtgcaaacacctgattgacatagctcactacaacccagaacttctggactcaagtgatcctcctgtcttagcctcctgagtagctaggtctacaggcatgtgccactgtgcctggcaaaaagtcttttttaagtgctaagaaaaaaaaaagagcaaatgatttgaacagatatttcaccaaagatatgagtgcccaacaagtacctgaatcaaaacttaatgttattgatcatcagagaaatgcaaattaaaaccatcaaattattactatatatccattagaatggctaaaactaaaaatattatcaaatgagggcaagaatatagcaattggaactttcattcatggtggtgagaatataaaatggtacaaccactttgcaaaaagcgttttggcagttttttttttttttttgagacggaatctcgttttatcacccagactggagtgcagtggtgtgatcttggcccactgcaacctctgcctcctgggttcaagggattctcctgcctcagcctcctgagtagctaggattacagatgcctgccaccacacccagctaatttttgcatttttagtagagacggggtttcaccatgttagctaggctggtctcaaactcctgacctcaagtgatccgcccacctccgcctcctaaagtgctgggattacaggtgtgaactaccacgcccagccccccagctcattcttagctaactagtgtgtgtgaaaaagagacagtgttaaaatatatatggtttaaactgataaggaaatgatcagttattgagcttatccatgattgctaattcaggtagagatggcttataagtaagtgttcggggctgcttacgggaagaaaaaatgaaagttagggatttcctttggatgctgggaaacaaaactccaactgggttctgacaaacataccatgtgcattgtcctgtggagacatgacaatgtaaacccataaacaaatcgattacgttttggtgacaactattgtgaagagaatggccatagtatttgctgcttctccttttaataggtagcatctctcctcttactcccttgaatctgagatagccttatgaagtgatattgtgccagttctgagactaggcctcaagaagcctcgaagcttccaatcttgcacttttttgtttgttttgatacaggtgcttgttctgttgcccagcctagagtgcagtggcacaatcatggctcactacagcctcaatctcatgggctcaagcaatcctcccatctcagcctcccaaatagctgggactacaggcatgcagcaccaccccaccctccccacccccagctaattttttaaaatttttttgtagaagaccaggcgtggtggctcacacctgtaatcccagcactttgggaggctgaggcaggcagatcacctgaggtggggaattcaagaccagcctgaccaacacggagaaacccatctctactaaaaatacaaaattagctgggcgtggtggctcatgcctgtaatctcagctactcaggagactgaggcaggagaatcgcttgaacccaagaggcaaaggttctggtgggctgagattgcgccattgcactccagcctgggcaacaagggcgaaactccatctcaaaaaatttttttttttacagatgggctctcactatgttgcccaggctggtcttgaactcctgggctcaagaaatcccccaaccttggcctcccaaagtgctgggattacaggtgtgagtcatcatgcccagccccaatctcatactcttgaaatcctaaagccatgtgaagaatccaggcctagcttgctggatgatgagagacacagtccccctaatgccccaggtgacagtcactcaataccagacatatgagtgacaccatctaggactagccagcctcaacaacccaactagtgacctcagctgcatgggcaagtccagccaagataagctgagctggatccagactataagaattacctggaagaacgcaaactaatgaaagattgttgttttaagccaatgagctttggggtgatttgttaattggcaatagataactgatattcaaggattcatccaaagttcccttaaaagatagaacccattaagtcattttaaacacttataagcaagttattaaatccttaaaagaaactgaaagtttctaaggtatactgggttggaaaaaggaaaagaaaaagaaactaaaagtgaaggctgaaactgacaagtaaggagttatttctccctgcaaatgtaatcagaaaataaggtggagtgtctctgaatgcataactggaacaaggaaacaatctaatggttttagtagtaaatatatgatttcaggggcacatccagtggaatgatggagtcagtgcacaacaacttgtaagacccagtcatggaaactggcaaacattacaagttagaaccagttgttaaatcttcattagtacatcactggacacatctattgctaaaggcacatttcatcagtatgtatatgcataaatatacatataagatgtccttaatgtttaaaaaagacattggttggttctgccacaatctgtgatcttgggcaagtcaattagtgtctttggatctgtttccaaatcagtccccaaaaatcatctttaagatgtctttcagctttacgattctatcttctatgctcttatggtaattacacctggatgcagcaattgaaaagtccaatgggatcaatccaaattgccacacttaaccatgttactgactacatatattactcatcaagacaattattcaagtaagtggcataatagtaatccaatgtactttgcattatgagtgaagaagagactaattttgactagaggggaaagaagggatggtcatagcaagatactttgtcaatcaggaatgagggctatctttgaacccacagtggcttgaactctataggtgcttaataaaatttgccgaaaagattacatgcttagagacaacattataaagaaaagacattcttggccgggcgtggtggctcatgcctgtaatcccagcacttcaggaggcgaaagcaggtggatcacctgaggtcaggagtttgagaccagcctgaccaacatggagaaaccccatctctactaaatacaaaaaattagccggacatggtgttgcatgcctatagtcccagctacttgggaagctgaggcaggagaatcgcttgaacccgggaggtggaggttgcagtgagctgagaatgtgccactacactccagccaaggcaacaagagcaagactctgtcccaaaaaaaaaaaaaaaaaaaaaagagacattcttgctgaattgaagactcagaagaggctgggcacagtggctcacccttgtaatcccagtattttggggggccaaggtgggcagatcacctgaggtcaggagttcaagaccagcctggccaacgtggtgaaaccccatctctactgaaaatacaaaaaatcagccaggcatgctggtgcacgctcataatcccagctactcgggaggctgaggcaggagaattgcttgagcctatgaggcggaggttgcagtgggctgagatcatgccactggccactgtactgcactccagcctgggtgacaaaagtgaaactccatctcaaaaaaaaaaaaaaaaaaaagactcagaagtaatcataaggttctacttgctattctcacatgtaattgtgagactctgcctccatttctccatctaaaaacaggagctcatttacaagcaacatgacaagaattcaagcagtcatggctgtgaagcatttctgcagaaggatatgctatgtaagtatgaggttgttactaaatcaaaatgaatgcctttgtgcaaaactagaaagcacattacatattgttcctgagtattccttcccagtgcattcaaaatattctcacattcacaaggttaaacagcacattaaaaaatagtaggaggctgatggctgagctcaattgggagtatctttctttggtgttagaatgtttgaaaattattttgggaagactatgagcaagttattttgaacttctggggaaaaaaaaaaatctgaagaagcattccctttgcctaaaagcaaaggagacatttatttatgcctttagcaaataaaatagtttgcttactaccagtgtttgtgggctgatattcaactcatcttctggaaattttaaaaatacacattgaaactgaaaaagtattctttgagtaagggtttacctgaagtgcccagaaccatccaaaatgatggcacattatatctttttttcttaaaaatttttggaatctaattgaagatgcctcttagaatatgtggaaaccacacgtgctatcttgcatatcactatcatttcagttctaatgttattaggtgtttagctacaggcaagtagaattagggcatgatgtgacagactgtaatgagttgctgagaaactacatactctatccccaggaaaacacatattctcaaaattctacacaatttcaggaatttcatagatgcccctaccccaaatcccattcatgaaatccttagcttaaaatcctgtgcactagagcaatgtattttataaaaccatattcagatgcctgtgaagcaatgaatgtgctaggcaatgttaggcggtagaaacagtgatacacgtagtcagacagggtacctagaagtcatggagcttataggctagtaggggatatggacatttaccaaataatcacacaaaaagatgcctaattacaaactctgattaagtgctatggagagatatacagtgttgcacgtaacaacagaatctaaagaagttacattttagggggcatataaacaatgttgtgcaggggaggtagaagaaacacattatggtaaagggctgcaaaggaaataagcccataataaggcctcttataggtttaagctaggacctgaaacttgtatactttatatgctttgaaatgagacatacattaaagtggctgatcaaattaaaacattttccagtctttgcctactaaattgataaagattttttaaaattttaatagaactaaagagaaaatatttctatatactgatgttaggagtatgcagtttaggccaggcatggaggctcacacctataatcccacccagcactttgggaggccaaggtgtgtggacacttgaggtcaggagttcgagaccagcctgaccaacatggtgaaaccctgtctctactaaaaatgcaaaattacctgagtatggtggtgcacacttgtaatcccaactacttaaggaggctgaggcaggagaatcacttgaacccgggaggtggaggctgcagtgagccaagatcgcgccattgcattccagcttgggcagagcaaacctccatctccaaaacccaaaaagtatacagtttaaaccactgactttaaaaatgtacataaacatggatgccggacatggtgattcaacgattgcacttacagaaacaaatctaagaaaacagtaatgatcttgccagcttctgatgagattataagaaaaaaaaaagaagaaataaatttaaaaaaaaaataaaaaaagaaaatggtaataatccaccaggatgttaataacagcattattcacaagatggaacagaaacaatgattttgtctaacagcagggagttaattaaattatgacaagccagattatagaataatatgcacccattaaatcagagtacttaatgatacggaaaaaattcctattaagtgaaaaaagcattacaaaacagcatatattatgagctctatttttatttttgaaatatatttatgcagagaaatacaaaatgttaacaatattatcttaaaaaaaaaaaataaggctgggcacagtggctcacacctgtaatcccatacttttggaggccaaggtgggtggatcgctttgagcccaggagttcaagaccagcctgggcaacatggcgaaaccccgtctctataaaaaaaattaaaacaattagccaggcatggtagcacacatgtgtagtctcagcaattcgggaggctgcggtgggaggattgcttgagcccaggatattgaggttgcagtgcaatgtgattgtgccactgcactccatcctgggcgacacagcaagaccttttctttaaaaaaaaaaaaaaatcagtttttgctattggtctactcagaatattccagcacttaatttcactattaccatttattctactagtcattctcaactaatgaacatccaaattctctgctaattaagtgcttttaaaagtcacttttgggcgagatgttcaaattaagccctgggtgagagtgccctctggtggtttcccaataatgcttgaacaagaactgtgtagtgagtttttcatgaagctaaatgtatttaaattaaagaagcatcccactttacgaattttaaaatgtctgcaaaacagacaaataagtagatctttcataaaatgttactgatggtggataacaggttcttatccctgggggacgggggaggaacagagggcaggtgatgctggtgatcacggactatgtgcttatttagcaaaattaaaaatcagcaacccatgaaaagcaaaatcccagaaagcacagtgttaatctatacttccagtagaataaagtcaaagttaattctccaaagcactgacacataagtatgtggatgtgggcatcttgggtaaatccttatttagcagagctttgtactcggaagagaagaaaatcttcataatcatattttgatttttcacttctttctacatttataacatagctaagaatttgtagaattttggatataagtcaacctgaaagaaaaccaaacatttttcaagaatacaccatcgacaaagctggtaaatatttctgatttatcaagttcaatcaaacttgtttttttaatctttccaaatgaaatttatattaatggaaaaagtaaaccacttaacagagggtcaccattattaattatttcctttactctctattcctcacacttcactggccacttgaaacttctagagttcctttattaaaataactagatcaaacaatagactttgagaaattatttttcatatcaattttacaaatactgtatcacaaacattctacagtacaaatttaaataaagcaactttctaccttattaaaagattcttcacctcctaaatagaaactgaaggggaagcaatgctattaaggatcatacataagctaatagaggcagcagaattatctattaacattttcctaacactattctagtgaccttaacattttaatcacagagctgcagctgtttgcatgtgttctaaagctagcataatctttaagacagtcaggaaaaaaaaccttcaaaacaaattacataatattctatctagaaaaatttccaggaaagcacattcttgggtgaaagaaaaccacccctttgtcattgtgatgcactaaaaaaaagctttggagcctgatagtttggctcctggctctcccacttgtttgggtaaggttcgagtcactgtaaaatgtaattatactcccttttcaaaggattattttgagaatttaataagaattgatggaaggggcctagcagatagtaaaacctgattaaaatatcactaatttaattatttcctagaagccaactgaaacatcataacatttattttcttggtagaccttatgagtttattctcaaaggcaattaaaaaatctccttcaggaaagccatgcacatttttattaatcatatttatactactaacaatgcttggctgatgattaaaaatacttaaatcacagtagacacacaaaaagagatgtttctcaacttatcatagggttacatcccaataaacctactatcagttgaaaatattgtaaattgaaaatgctagcctgtcttaaatatgctcagaacacttacagtagcctactgtttagcaaaattatctaacacgaagcccgttttataataaagtgttgaatttctgatgtaatttattgatgttctactgaatatgtatggctttggcactatggaaaagtcctaaattggagaccgcacataaatgaaacactaaaatagaaaaagaaaaaagaaaataggtttctctaaatgagaatgtcaaatccagaattactttatataaaagtacacattctaatatatgaaaagatattttatcattattactttactatatattactgaatacaccagactgcattttctcaaatggcaaatgaggcacatttctctttgattcccccaggaacctccgcatcatctgtcttttggaggattcagattcttacgacatctgtgataccgtccatgaggataccaacggtgcttagtagtaaagaacattttgctaagttgttctatcataggtccttcctcaaggtgttcaactttttcttccaatctggttttcagcacttgatcatgtgtttcttcattattatgcacaggatctggccgagggataggttttgtgtgttcatatggaatgtccacagaagggtggtagcatactattgtcctgccatcagaagtcagagcaagctctacgttgcaattatagtcatctggtagaggagaatacgtagatttatgacaaacacaatataaagctccattttggactggaaataaatgtttcaagatagttctctttgacatcacccattttactgcagctacagccatggtgtttcaagatgcttatcaagtggtatgaaaaaagatgttctgaagagaaactgcttttagaatctgcttctaagcataccaatttctactcctgcttgacggcttctcaccacgaacccgccatcttgtttcaat

SEQ ID NO: 14003 - RNA, 11547 nt, Homo sapiens
  source 1..11547: mol_type = other RNA
gctgggattacaggcatgagccaccgcacccagcccaatgtatatctttataaagctgggaccaaactggcttcttgcagcaataattaaatgttcaaatatgctcaacagaactttccctctagataatcatcatatctctaaatgtaatcacagttgtttgttttccaaactattacataaagagaacaatctcaaacttattgcattagcctttacacaagttatgttctttactaagtcactgaacacactgtacagttcagttgatatgctttttctaccaagactttttcaaataaaaagatatagtaggttgatttacattctagggcaagctccttaatttaggtaattattccggaatgttctcttaccactgctgctatccatccaattggattcctacaaagcttcaaaccacattaattaacaaagtaatttattccacactttactgttgtttagagttagctgtttgttggcaatgaagtggaaaaaagagaatcttccttcatattactatcatattcaaatagcatataaactaattgccatattagtaatatctatatattaatggtacatcaaaccaattgcaagaaaaggtaatttattagctttctttgttctatgggttgatcttcctggatatttcaaattgttgtgtgttggtaactggtaattgaagtactttctttgccacacagtctcccaacatttctaagaatctttgatgctgattattattaagacaattattgtctatatataagattattgtcttaattgcattttttagttttagcaatctaaagttgcttaaagatgtctaaaaagcattaacgtttatttgtgaaataatgaatatctgtgctttcagttttttaattacttaggtttttctttcaaagagatcttctggttttggatttatctctttatgttctgtatttaaatgttgatttagttttgattattttattgcttcatttgccagaacttctcagcaaataacatgttatggttttcccatgtcttcatttatggctaaaaaactgaactcagtatatgaagaattatatttatgagtaaaactagaacaatctattggttttcatttattcagaatcgcttttattgtcaccattaggtttactaatactgttgcattcagaaaaggtaagtcttttcttgataaaaaaagccagtgaagttattttgccatccataacatggtgttaaagataaatgaaacaaattaccccaaaccttcacatcgattgcattccctgcctgaaactttctctcctttctctttaaacagatctaatcttaacactggtcccccataaaaatatttccagtgcatatatctgacaaaagatttatccaaaatatttaaagaaatattataacttcaatcataagaagaaaaaataatgagtaaatagatgttccatatcacatattatcagggaaatgcaaattaaaataaatgtgatgtggatgagctgtctgagcagagaaaaacacaaaacaagtgagacaccactacacaccttttagaatggccaaaattcagaacactaacaccaagtgctgacagggatgttgagcaataggaacccttattcactgctggtgggaatgcaaaatggtacagcctctctgtaggacagtttggtggttttttacaaaacgaaacattctcttagcattcaatccaacaattgtgctctttggtatttacccaaaggagttgaaagcttaaatggacacaaaaacctacacatggatatctatagcaattttattcataattgccaaaacttggaagcaatcaaccaagatgtccttcagcaggtgaatggataaactgttgtacacccagacaatggagtattactcgatgctaaaaagaaatgagctatcaaactgtgaaaagacatagaggaaacaaatgcatattatccagtgaaagaaaccaatgtgaaaaggctatatatactttatgattccaactatatggcgttctgaaaaaggaaaaacttacggagacagtgaaaagaccagtggtagccgggggtcagtggggaggacacgacgaagaggcagagccaagggtttttaggacagtgtagactctgcatgactataaagatggatacatgtcattgtacctttgttcaaacccatagattgtacagcaccaagagtgaaccctaatggaaacaataggctttgggtgataatgatgtgtcagtgtaggtttatcaattgtaaccaatgtgccactctgctgggggatggtgatgagggaggcatgggggaggggagcactgaggatatataagttatttctgtaccctcctctcaattttgctcagaacctaaaactacttttaaaaactaaagttttttttttttttcaggagatgaggatctcactatgttgcccaggctgcagtgcagtggctattcacaggtgtgatcccactactgatcagcacaggagttttgacctgctccacttctgacgctccttaggcaactctgggtcccagtgacccaggaggtcactacatttatgctgaacttagtgcaaacacctgattgacatagctcactacaacccagaacttctggactcaagtgatcctcctgtcttagcctcctgagtagctaggtctacaggcatgtgccactgtgcctggcaaaaagtcttttttaagtgctaagaaaaaaaaaagagcaaatgatttgaacagatatttcaccaaagatatgagtgcccaacaagtacctgaatcaaaacttaatgttattgatcatcagagaaatgcaaattaaaaccatcaaattattactatatatccattagaatggctaaaactaaaaatattatcaaatgagggcaagaatatagcaattggaactttcattcatggtggtgagaatataaaatggtacaaccactttgcaaaaagcgttttggcagttttttttttttttttgagacggaatctcgttttatcacccagactggagtgcagtggtgtgatcttggcccactgcaacctctgcctcctgggttcaagggattctcctgcctcagcctcctgagtagctaggattacagatgcctgccaccacacccagctaatttttgcatttttagtagagacggggtttcaccatgttagctaggctggtctcaaactcctgacctcaagtgatccgcccacctccgcctcctaaagtgctgggattacaggtgtgaactaccacgcccagccccccagctcattcttagctaactagtgtgtgtgaaaaagagacagtgttaaaatatatatggtttaaactgataaggaaatgatcagttattgagcttatccatgattgctaattcaggtagagatggcttataagtaagtgttcggggctgcttacgggaagaaaaaatgaaagttagggatttcctttggatgctgggaaacaaaactccaactgggttctgacaaacataccatgtgcattgtcctgtggagacatgacaatgtaaacccataaacaaatcgattacgttttggtgacaactattgtgaagagaatggccatagtatttgctgcttctccttttaataggtagcatctctcctcttactcccttgaatctgagatagccttatgaagtgatattgtgccagttctgagactaggcctcaagaagcctcgaagcttccaatcttgcacttttttgtttgttttgatacaggtgcttgttctgttgcccagcctagagtgcagtggcacaatcatggctcactacagcctcaatctcatgggctcaagcaatcctcccatctcagcctcccaaatagctgggactacaggcatgcagcaccaccccaccctccccacccccagctaattttttaaaatttttttgtagaagaccaggcgtggtggctcacacctgtaatcccagcactttgggaggctgaggcaggcagatcacctgaggtggggaattcaagaccagcctgaccaacacggagaaacccatctctactaaaaatacaaaattagctgggcgtggtggctcatgcctgtaatctcagctactcaggagactgaggcaggagaatcgcttgaacccaagaggcaaaggttctggtgggctgagattgcgccattgcactccagcctgggcaacaagggcgaaactccatctcaaaaaatttttttttttacagatgggctctcactatgttgcccaggctggtcttgaactcctgggctcaagaaatcccccaaccttggcctcccaaagtgctgggattacaggtgtgagtcatcatgcccagccccaatctcatactcttgaaatcctaaagccatgtgaagaatccaggcctagcttgctggatgatgagagacacagtccccctaatgccccaggtgacagtcactcaataccagacatatgagtgacaccatctaggactagccagcctcaacaacccaactagtgacctcagctgcatgggcaagtccagccaagataagctgagctggatccagactataagaattacctggaagaacgcaaactaatgaaagattgttgttttaagccaatgagctttggggtgatttgttaattggcaatagataactgatattcaaggattcatccaaagttcccttaaaagatagaacccattaagtcattttaaacacttataagcaagttattaaatccttaaaagaaactgaaagtttctaaggtatactgggttggaaaaaggaaaagaaaaagaaactaaaagtgaaggctgaaactgacaagtaaggagttatttctccctgcaaatgtaatcagaaaataaggtggagtgtctctgaatgcataactggaacaaggaaacaatctaatggttttagtagtaaatatatgatttcaggggcacatccagtggaatgatggagtcagtgcacaacaacttgtaagacccagtcatggaaactggcaaacattacaagttagaaccagttgttaaatcttcattagtacatcactggacacatctattgctaaaggcacatttcatcagtatgtatatgcataaatatacatataagatgtccttaatgtttaaaaaagacattggttggttctgccacaatctgtgatcttgggcaagtcaattagtgtctttggatctgtttccaaatcagtccccaaaaatcatctttaagatgtctttcagctttacgattctatcttctatgctcttatggtaattacacctggatgcagcaattgaaaagtccaatgggatcaatccaaattgccacacttaaccatgttactgactacatatattactcatcaagacaattattcaagtaagtggcataatagtaatccaatgtactttgcattatgagtgaagaagagactaattttgactagaggggaaagaagggatggtcatagcaagatactttgtcaatcaggaatgagggctatctttgaacccacagtggcttgaactctataggtgcttaataaaatttgccgaaaagattacatgcttagagacaacattataaagaaaagacattcttggccgggcgtggtggctcatgcctgtaatcccagcacttcaggaggcgaaagcaggtggatcacctgaggtcaggagtttgagaccagcctgaccaacatggagaaaccccatctctactaaatacaaaaaattagccggacatggtgttgcatgcctatagtcccagctacttgggaagctgaggcaggagaatcgcttgaacccgggaggtggaggttgcagtgagctgagaatgtgccactacactccagccaaggcaacaagagcaagactctgtcccaaaaaaaaaaaaaaaaaaaaaagagacattcttgctgaattgaagactcagaagaggctgggcacagtggctcacccttgtaatcccagtattttggggggccaaggtgggcagatcacctgaggtcaggagttcaagaccagcctggccaacgtggtgaaaccccatctctactgaaaatacaaaaaatcagccaggcatgctggtgcacgctcataatcccagctactcgggaggctgaggcaggagaattgcttgagcctatgaggcggaggttgcagtgggctgagatcatgccactggccactgtactgcactccagcctgggtgacaaaagtgaaactccatctcaaaaaaaaaaaaaaaaaaaagactcagaagtaatcataaggttctacttgctattctcacatgtaattgtgagactctgcctccatttctccatctaaaaacaggagctcatttacaagcaacatgacaagaattcaagcagtcatggctgtgaagcatttctgcagaaggatatgctatgtaagtatgaggttgttactaaatcaaaatgaatgcctttgtgcaaaactagaaagcacattacatattgttcctgagtattccttcccagtgcattcaaaatattctcacattcacaaggttaaacagcacattaaaaaatagtaggaggctgatggctgagctcaattgggagtatctttctttggtgttagaatgtttgaaaattattttgggaagactatgagcaagttattttgaacttctggggaaaaaaaaaaatctgaagaagcattccctttgcctaaaagcaaaggagacatttatttatgcctttagcaaataaaatagtttgcttactaccagtgtttgtgggctgatattcaactcatcttctggaaattttaaaaatacacattgaaactgaaaaagtattctttgagtaagggtttacctgaagtgcccagaaccatccaaaatgatggcacattatatctttttttcttaaaaatttttggaatctaattgaagatgcctcttagaatatgtggaaaccacacgtgctatcttgcatatcactatcatttcagttctaatgttattaggtgtttagctacaggcaagtagaattagggcatgatgtgacagactgtaatgagttgctgagaaactacatactctatccccaggaaaacacatattctcaaaattctacacaatttcaggaatttcatagatgcccctaccccaaatcccattcatgaaatccttagcttaaaatcctgtgcactagagcaatgtattttataaaaccatattcagatgcctgtgaagcaatgaatgtgctaggcaatgttaggcggtagaaacagtgatacacgtagtcagacagggtacctagaagtcatggagcttataggctagtaggggatatggacatttaccaaataatcacacaaaaagatgcctaattacaaactctgattaagtgctatggagagatatacagtgttgcacgtaacaacagaatctaaagaagttacattttagggggcatataaacaatgttgtgcaggggaggtagaagaaacacattatggtaaagggctgcaaaggaaataagcccataataaggcctcttataggtttaagctaggacctgaaacttgtatactttatatgctttgaaatgagacatacattaaagtggctgatcaaattaaaacattttccagtctttgcctactaaattgataaagattttttaaaattttaatagaactaaagagaaaatatttctatatactgatgttaggagtatgcagtttaggccaggcatggaggctcacacctataatcccacccagcactttgggaggccaaggtgtgtggacacttgaggtcaggagttcgagaccagcctgaccaacatggtgaaaccctgtctctactaaaaatgcaaaattacctgagtatggtggtgcacacttgtaatcccaactacttaaggaggctgaggcaggagaatcacttgaacccgggaggtggaggctgcagtgagccaagatcgcgccattgcattccagcttgggcagagcaaacctccatctccaaaacccaaaaagtatacagtttaaaccactgactttaaaaatgtacataaacatggatgccggacatggtgattcaacgattgcacttacagaaacaaatctaagaaaacagtaatgatcttgccagcttctgatgagattataagaaaaaaaaaagaagaaataaatttaaaaaaaaaataaaaaaagaaaatggtaataatccaccaggatgttaataacagcattattcacaagatggaacagaaacaatgattttgtctaacagcagggagttaattaaattatgacaagccagattatagaataatatgcacccattaaatcagagtacttaatgatacggaaaaaattcctattaagtgaaaaaagcattacaaaacagcatatattatgagctctatttttatttttgaaatatatttatgcagagaaatacaaaatgttaacaatattatcttaaaaaaaaaaaataaggctgggcacagtggctcacacctgtaatcccatacttttggaggccaaggtgggtggatcgctttgagcccaggagttcaagaccagcctgggcaacatggcgaaaccccgtctctataaaaaaaattaaaacaattagccaggcatggtagcacacatgtgtagtctcagcaattcgggaggctgcggtgggaggattgcttgagcccaggatattgaggttgcagtgcaatgtgattgtgccactgcactccatcctgggcgacacagcaagaccttttctttaaaaaaaaaaaaaaatcagtttttgctattggtctactcagaatattccagcacttaatttcactattaccatttattctactagtcattctcaactaatgaacatccaaattctctgctaattaagtgcttttaaaagtcacttttgggcgagatgttcaaattaagccctgggtgagagtgccctctggtggtttcccaataatgcttgaacaagaactgtgtagtgagtttttcatgaagctaaatgtatttaaattaaagaagcatcccactttacgaattttaaaatgtctgcaaaacagacaaataagtagatctttcataaaatgttactgatggtggataacaggttcttatccctgggggacgggggaggaacagagggcaggtgatgctggtgatcacggactatgtgcttatttagcaaaattaaaaatcagcaacccatgaaaagcaaaatcccagaaagcacagtgttaatctatacttccagtagaataaagtcaaagttaattctccaaagcactgacacataagtatgtggatgtgggcatcttgggtaaatccttatttagcagagctttgtactcggaagagaagaaaatcttcataatcatattttgatttttcacttctttctacatttataacatagctaagaatttgtagaattttggatataagtcaacctgaaagaaaaccaaacatttttcaagaatacaccatcgacaaagctggtaaatatttctgatttatcaagttcaatcaaacttgtttttttaatctttccaaatgaaatttatattaatggaaaaagtaaaccacttaacagagggtcaccattattaattatttcctttactctctattcctcacacttcactggccacttgaaacttctagagttcctttattaaaataactagatcaaacaatagactttgagaaattatttttcatatcaattttacaaatactgtatcacaaacattctacagtacaaatttaaataaagcaactttctaccttattaaaagattcttcacctcctaaatagaaactgaaggggaagcaatgctattaaggatcatacataagctaatagaggcagcagaattatctattaacattttcctaacactattctagtgaccttaacattttaatcacagagctgcagctgtttgcatgtgttctaaagctagcataatctttaagacagtcaggaaaaaaaaccttcaaaacaaattacataatattctatctagaaaaatttccaggaaagcacattcttgggtgaaagaaaaccacccctttgtcattgtgatgcactaaaaaaaagctttggagcctgatagtttggctcctggctctcccacttgtttgggtaaggttcgagtcactgtaaaatgtaattatactcccttttcaaaggattattttgagaatttaataagaattgatggaaggggcctagcagatagtaaaacctgattaaaatatcactaatttaattatttcctagaagccaactgaaacatcataacatttattttcttggtagaccttatgagtttattctcaaaggcaattaaaaaatctccttcaggaaagccatgcacatttttattaatcatatttatactactaacaatgcttggctgatgattaaaaatacttaaatcacagtagacacacaaaaagagatgtttctcaacttatcatagggttacatcccaataaacctactatcagttgaaaatattgtaaattgaaaatgctagcctgtcttaaatatgctcagaacacttacagtagcctactgtttagcaaaattatctaacacgaagcccgttttataataaagtgttgaatttctgatgtaatttattgatgttctactgaatatgtatggctttggcactatggaaaagtcctaaattggagaccgcacataaatgaaacactaaaatagaaaaagaaaaaagaaaataggtttctctaaatgagaatgtcaaatccagaattactttatataaaagtacacattctaatatatgaaaagatattttatcattattactttactatatattactgaatacaccagactgcattttctcaaatggcaaatgaggcacatttctctttgattcccccaggaacctccgcatcatctgtcttttggaggattcagattcttacgacatctgtgataccgtccatgaggataccaacggtgcttagtagtaaagaacattttgctaagttgttctatcataggtccttcctcaaggtgttcaactttttcttccaatctggttttcagcacttgatcatgtgtttcttcattattatgcacaggatctggccgagggataggttttgtgtgttcatatggaatgtccacagaagggtggtagcatactattgtcctgccatcagaagtcagagcaagctctacgttgcaattatagtcatctggtagaggagaatacgtagatttatgacaaacacaatataaagctccattttggactggaaataaatgtttcaagatagttctctttgacatcacccattttactgcagctacagccatggtgtttcaagatgcttatcaagtggtatgaaaaaagatgttctgaagagaaactgcttttagaatctgcttctaagcataccaatttctactccttgacggcttctcaccacgaacccgccatcttgtttcaat

SEQ ID NO: 14004 - RNA, 1429 nt, Homo sapiens
  source 1..1429: mol_type = other RNA
gctgggattacaggcatgagccaccgcacccagcccaccaagatttttatagattaaattctatttctaagatctgctccaaaattaattcaataagacaaagtagaagtaggtaagattagtcataaatagttgatgctgggtaatgatacatgggagttcattagactagcctgtctacttttgttttacgtaaaattctccataataattttaaaaagttacgtttgtttttgtagtcctcaagaggggatgttcactaaggtcacagcaaagttgcactatacgactctggcttatacccagaaagcatctagccaaacctagcctaagttatgctagattctgaggtcttgctacgacagaaggaagggaagaccacagtggttgtagacttcagagaaataattctttttttttttttttttttgagacagagtctcgctctgtcacccaggctaaagtgcagtggcatgatctcagctcaccacaacctccacttctcaggttcaagcgattcccctgcctcagcctcctgagtagctgggattacaggcgtgagccaccatgctcagctaatttttgtgtttttagtagagacagtgtttcaccatgttggtcaggctggtctcgaactcctgacctcacgtgatccacctgcctcggcctcccaaagtgctgggattacaggcatgagccaccgtgcctggcctaaaataattctttttaaggcccttctacaacaccccaaatgtagaactgagttgctgtattaaatttgacatttaaatcttggttaaaacaacaacaaaaaaagggataaagaatatttactgtgttttttgctttatttattcagagagtgaaactgtgttacagtgagctaaatttttagctgtacttagaatgtgctccctcctacatttcactctggaaaagtgaagtatcttatcatttcttagaaacctggatgtgaaactagtcaatattaagatcttatacacatcctgagtgatgcccaatttaaggctttgaatagctattcatgtaagttgacttttctgtgcatttgtatcggggaggatccagttcaggttgatgtcctgggaaccagtgaggctctcgcttaaatcctgggaaggcaagggtttgggctgcacgatattcctcaggtcatatctttcctggttccagttgcccatcagggtacggtttgaataggtattctcattagtggtgcatcgccatccatactggaaaaacttggacatattattccaatctgtccacacttcaccatggccatctgcattaacaaggctgccacagtgtgggtttgtgaggaaacaggcgaggttctgtctctggaagagaaattttgagcagcagagacactgggaggcagccatttcagacgaggtgaaaaaag

SEQ ID NO: 14005 - RNA, 1496 nt, Homo sapiens
  source 1..1496: mol_type = other RNA
gctgggattacaggcatgagccaccgcacccagcccaccaagatttttatagattaaattctatttctaagatctgctccaaaattaattcaataagacaaagtagaagtaggtaagattagtcataaatagttgatgctgggtaatgatacatgggagttcattagactagcctgtctacttttgttttacgtaaaattctccataataattttaaaaagttacgtttgtttttgtagtcctcaagaggggatgttcactaaggtcacagcaaagttgcactatacgactctggcttatacccagaaagcatctagccaaacctagcctaagttatgctagattctgaggtcttgctacgacagaaggaagggaagaccacagtggttgtagacttcagagaaataattctttttttttttttttttttgagacagagtctcgctctgtcacccaggctaaagtgcagtggcatgatctcagctcaccacaacctccacttctcaggttcaagcgattcccctgcctcagcctcctgagtagctgggattacaggcgtgagccaccatgctcagctaatttttgtgtttttagtagagacagtgtttcaccatgttggtcaggctggtctcgaactcctgacctcacgtgatccacctgcctcggcctcccaaagtgctgggattacaggcatgagccaccgtgcctggcctaaaataattctttttaaggcccttctacaacaccccaaatgtagaactgagttgctgtattaaatttgacatttaaatcttggttaaaacaacaacaaaaaaagggataaagaatatttactgtgttttttgctttatttattcagagagtgaaactgtgttacagtgagctaaatttttagctgtacttagaatgtgctccctcctacatttcactctggaaaagtgaagtatcttatcatttcttagaaacctggatgtgaaactagtcaatattaagatcttatacacatcctgagtgatgcccaatttaaggctttgaatagctattcatgtaagttgacttttctgtgcatttgtatcggggaggatccagttcaggttgatgtcctgggaaccagtgaggctctcgcttaaatctatgtgttgaaagtggcattttgttgttgtagcttgtatcatatgttgtttcaaagtagtgtccaaactgggaaggcaagggtttgggctgcacgatattcctcaggtcatatctttcctggttccagttgcccatcagggtacggtttgaataggtattctcattagtggtgcatcgccatccatactggaaaaacttggacatattattccaatctgtccacacttcaccatggccatctgcattaacaaggctgccacagtgtgggtttgtgaggaaacaggcgaggttctgtctctggaagagaaattttgagcagcagagacactgggaggcagccatttcagacgaggtgaaaaaag

SEQ ID NO: 14006 - RNA, 2659 nt, Homo sapiens
  source 1..2659: mol_type = other RNA
gctgggattacaggcatgagccaccgcacccagcccacttcaatattttcatcagtaaattagtatactttagagttgtggtgattaaaataatatatgtaaagcatataagtagaatgcttggcaaacagcaagtgcttactaagcgttagctactcataatagtaacagctgatttaataataggatctgtaaataagatagtattttctgctctacaaatgaagaaattaacacgtacagaggataagttaatttgcctaagattgtccagctaaataaaaagtagagccagattgaacccaagaagtataacttcagagatcaatctcttaactgcaatactattacactcccttattattcattcatttatttcacaaaaaattaactgccaggtactgtttgtcactaataacattatttatattgaatacagaagaaaatatgcacaatgtgatgaagatgggcatataatgacatagctttttactttgacaaagcctaatccaaatatttaagcatttttataagtatcatctgctttaaaaatatagtcaatgaatattgcttctccccaataacatgagccagataatttcaaataaataatatgtttataaaaccttggatttttttcactgtattattcatgcatttaggtaagatgtgaatgaggatatttcttatttatttttttacttatttttatttttttgttttgttttatgagacagagtctcgctctgcctcccaggctgtagtgcagtggcacgatctccgctcactgcaacctccgtcccgggctcaagcgattctcctgcctcagcctcccgagtagctgggattacaggcgcccaccaccatgtccagctgatttttgtatttttagtagagacagggtttcaccatgttgcccaggctggtcttgaactcctgacctcaaaatgatccacccacctcagcctcccaaagtgctgggattacaggcgtaagccactgtgcccagctacttatttttaaagattttaaaattaccaataaacactagccatagattgacccttgtattctaactaccagaaagcagacaagtcataaaccatttgcttctttatcctagtcatgaaataacgtgttctgaacagaagcactgacagttgagtttaaacagaaaacagcctgttagtttcatatgagtgggatcctttcaatatgcttaatttttgcttctgaaagtttctgccatctcaacgttcagtataactgttttttgagttttatgaatatatgtttatttatttttaaaaaccaaagagattttcttggtgattattgtcaaccaagctgtgacatgttaatgatgtagtttagtgtccctaataaagtcacatgaatgcttttcttaatattgtggggttttccattcaaaagtcaaccatatgattgcatatgtgctgaattagactttgtaaagagattatatagtgtcttcttgaatgttttatctaataaaagaaatataatggggtctgtgctacttctggccgaagcaagacaggtgagaatgttttttgtttctattaaataattcaattgctgacagttatctctttggtgtagaacataaaaaatgggtttaaaaatactataaggaaggaagcaaactattagtagaatctggatgaccaaaagatgtcttttcacagaactgtaagtcaaatctttctccataatggacgtacaggttcttatttttctcagatggcttacaaaagagtagtatgatgttagtactactaaaaaggaaaatccaataaatgtggttccaatgagacctgcaatctgagagatcatggctcctagttccatctgccgattgtagcataggctctcttctccttctgtagcctctatgactgagtagtatacggtaactggaatgattatgcccagtacaactccccatatgtaaatgcatagttttctagcaaagttgggctggcgaaattttttcagtaaatggccataaaatattttctcatagcatgaagtagtctcttgcgaggaatccttttgcattaaggtagcatagcggcttatggcaatccaacttaaaattaagagactgacaaacatacttgcatgcatggatagagttcccagaaaattgaccactctgcattgagcagattgatattcccattggaaacctttcaggaaatagatactcatgaaaggcatggcactgcacacaagtaagtttgcagtcacaaggtgtgacaggtagatgtgcgttgatgtttttttacctatttttgttaaaaatatccattgagagagagtgtttccaaaaacaccaacaatacaaaggaggatgtaaatgattggtaaagccatggaagagatcatagatggttgaatacatgttgtattgttgttcatttatgtcaggttttcttgaattttgtcacaggagcttttctaatcacgattgtccggttgaaataaagacaaaaagttacttattgtgatggataatgcctttgtctgtatgagtagtttatgccaactaaggttatattgttcagggcagtgatgccaaatttcagacttaaaattctctgatcttcactcttccaatatctttagtcagtgt

SEQ ID NO: 14007 - RNA, 4722 nt, Homo sapiens
  source 1..4722: mol_type = other RNA
gctgggattacaggcatgagccaccgcacccagcccaggcccgtctttcctctcctagtctgccccaatcggaaggatcaggaggcgtaaagctggcccatggggaacctgtggctgggagcccatgaggcaggggcagcagaagagggcagagacggttgggacctctgtggccctggctgaggtctgctctgatggcatggtaatggaaacctgctaccagatgacaaaacactattaccaaacagctgggtgaccttaggaaaatcactcaaccgctcctgcctacggatttcctcatctgcggggccctgcagagctgttgcaaggatgaaatgaggcaacgtacatgtgcctggcagcacagctgaccccacacagctcaatcctcagtgtttgcatgtttgggaaaaaaaaacaacaactagaggaactagttcttcttacctgggaagattcctaagcacaaattaggtttcttaggggctgagattagaaaaaacttggtctcagaccctagaccttattagcaggcccttcctagagctggctctaatcggcacagcttgggaagctctccacctggccactgctgtctttctgtttctggcttaggcccactggcctgcctggcgtgagctccctggggcagggagcttgcaaaccttgggagttgagaagcgctggctcggccaggtgtgggggctcacaccagtaatcccaacactttggtgaggctgaggcagaagagtcatttaagcccaggagttcgagaccagcctaggaaacagggagatcctgtctgcaaaaaatacagtggtgactcacacctgtagtcccagctactcggaggcaggctgagatgggaggatcacctgagcctgagaggcagagtctgcaatgatccctaatcacaccactgcactccagagcgccagagtgagatcctgtctttaacccctccccgaaaaaaaaagaaagaaaagtactgtccaacaggtcaggtccacactctagcttcagccttcttcctaaatcactgagtggccttgggcaaggccagaccctctctgggaagcagaaaggagatttttcccctgcctcctgggcagagattctggagagcactagtgtgtctgggtgagaaggaactctgtagctctacagtgccgggttctgtctggaagccttcttggggcctatgaccctgctatggtttgaatgtttgtcccctcccacgctcacgttgaaatgcgattgccactgtaacagtataagattagaccctaagaggtggtcaggccacgagggctctgccctcctgcgtggactcaggccgttatcttgggagtgggttcgctctctcccctcactcctgtcactctgtcctctgtcatgggaagatgcagaagggtcctcactgggctctgggccctccactatggacttcccagcctccagagctctgagccaatacatttctgtttattataacttaccccgtctcagggatcttgctagagcagcaaaaacagactcagacagaccctcacccccaggagcctgctcccaaccggggcccaaaagaaaacaagccagcgagggcactgcggaatgcagggttttggcgacagagctacaggagtgtgccttggcccccacaagggccacagtcctgcccccacctggtctcccggggctcagacagcagccgccagcccacggaggtagtcccccgccaggggcagcacggcccagtcatcggtccgcagggccacaggcactccatctgccagggccgcctccagccgcagcagcagctttgagtccgggggcaggtggattgctacacagtagctggtaggaggctgggccaccaccacaaaaggctccaggtggcgggacaccaagccctccaggccctgtggcccaagtggacaccacacacgactctcagcaccctctggcaggcaggaatcccagagctcctcaaagaagcccagcccggccccctctggaggctgcgggaaaggcagaaagaggtcggcaaagttcacgaacaggggtggcaagtgggcatggcacgtgagaccagtggatgtggtgtaaagggcatggacatccagccgtgcgggggccgggcatcggggctgcagaggcaggagcagagggcgggcagggcggccaggacacaggcagggcacatggacagcctccaggggtgcatacagctgtccttccacacggaagcgcagctccagagagtagatgggctccagcgcctccggctggagcttcaacactgggagtgggcccttgacccgatgggaccccaggctcagccgtaccagggccggtgcctcctgcaccatcagtgctgccacaaagccctggttctcggccaccagtgaagaggccagtgcaggtgcggcaagcgaggggcccagggccacccccaacttgggtgctgccaggtgtgccagcaggatgtagtagaggcgggcgtggtcacgcccatcagggtcctccagctgcctggccagcacctgcagcaagtcgaccaggccgcccctcacccctgcccgcagcagcgcccggcagacccgcagcaggccctgctgtaggtcccagttcgtgcagtgggcagccgcggcctgtagaaagttgagggtagcactctgggcatctccatctgccacctttgccagcatttgcaggtgccagcaaagagcttcatccctgcccggcctggacaccaccacctgccgcaacaccaccttcaggggctccctcagctcagagtccacctgatccaagaggtccacaaagtggggagccagcatgggccgggcttggtacagctgggccagtccgtggatcaagggggtcagcaccgtaggttgcccagccaggcagcaggccaccagatacgaggcctggaagcagagagtggccaaggcccgggggcccccatccagggctgcccgctgccgcaagccagccagcagctcttccaggtagtgccgtgggcttggaagctggcctttctcctcttcttcctcctcggcacagagcaggcacagtaaatgcaggcgggccaggagggccattgggtcatgcaggagactgggcaggagaccacggcatagctggggccctagcagcagtggggcagcctcctcaccttcagggcccagcggccagttctcagggaagctcaggacgcagtgaaggtaaaagagatgggtgggcggaggcagagcagggtgctgggcagccaaggtgagccggcggagcagcaacgcttcatcctgggctgtgaacaaggcctcaccaaaggccgccttgagcgcaagcatggcgtgcaacagtgtcagctgtgctgtgcctagcagccgtaccagctgcggcttgaagagtgccggtggctgtccctgcagaccccgcagggcccagcccagcagccacaggagctgggcctgggccacaggagtgagcagataggaggtgtccagaagctggatcaccgcagcccgcagctcccgcgcctcctcagggctgtgctctcgtgctgtaaggctacgctccccctctccctcctcagctgccggccagctgggtgcctggggctgaaggcgtccatcgccctcctccactagtgtccaatcccagggaccacccccagttggggagaccttatccgtgagcagtccccccaggccagccccaacccgggactggagcaccaaggtgttgcgcaaagcgagggccagcaacaggctgagtggctggacagggccttcctgccccagcaggccccgcagcaaccccagggagccccccagcagcccgggcttgcagctctctagctctcgcaggcactcgcaggccgtggcctgcaaggggcgctgttccgaggcggggacaaagcctcgccccagatcgctacccgcggccaggccgagcagtaggggcaggagccggcaggaggcgcccgaggtggggcccagcgcgccgcccgccgccagggcagtggtggccgccagcagcagtggccgacggagagctgagggccgcgggggtaggaggaccaaggtgtccaacagggaggtggcggccacttcggccgcagaggcgtcgggccacagctgcgcagggtactccatgctcagggccagcagggaaaccttggtctgttcgctcagcttctcacttctcaggtcgctcagcaggtcgcgacccaaatcctccccctcgggacctgccatgaaggcagacgggctggcccggaaggcccccaagcgctgggcccaggcgtcccggctcaggggccccatggtgaggcgcgcgggcccctgcgcagggaagagggaccctcaggccgcagccaccgggagcgcggggcccgctgccgaccccgaggggctgcggtcacccccagacgccgcgcagatgccggcgggacccgcgcccggctcccacggtgagaccagggctctcggggccgacgccagagctgggcgccggggccctcgcgggacaggacaggagcagggcgggggagggtgcgtgccgagagctcgttaggccgcctccctcccgcccgcggcccgcaccgaaaccacagcgccaccccggcccccggcgccggcggtaacgggccgcgctcgccgcctgactcagccgccgcgggcactcaggccggccggctccttccgggct

SEQ ID NO: 14008 - RNA, 6034 nt, Homo sapiens
  source 1..6034: mol_type = other RNA
gctgggattacaggcatgagccaccgcacccagccctaactattttttgtggaccaagaatgtacaagatgcttaacatatatgatctgtaattctcatattagccttgcaaaatagatatgaatacctccatttcacaaataagtaaaacaagaaattaagtaacttacccaaagtcacacaattattacagattcgggtctgtctggattcagatcttgtattctttttattattcaatgacaaattctcaaccaaaaggattatatgatttctaaaggtgtctcactaaaaactacaggcatgttgagtcagagggaaaatatggttgaatgttttggatctgacattttcttaaaagccaacactggtaactgttttcatcttcttccggcatcttaaggaatcacagaaacacatgtgagtcgggggtggttttgttttgtatactgcagccattactcattttttgggacatactcaatgcatactggatttggatccactgggctttgtcaaacacaggtgctcatgcattgattcaaatttgggttggcagagtaaatattcaatacggaggttcacatctctaaaagcgtatggaaagtatattaagaactacaatacataagaggggaatggggaaatcttctccctattgactagaggcctctcagatcaaggcttttttctccatttccagggtcactgactcaggccaggcccttattatctctcatctttaatgctacaatagcttcccaactatctgctgtgcctcaggcctctaccctaatctattccattttccacatcctccccagggttatgtccttaaaaatagttctgtcatgtctttttcctgtttataaaccactgccaatttccattgctcaaaagatcaaattaaaatcctgtcacatggcatacaaaacactttactatctggtattaatttctcattctagtctcatctcctttcctttctctgtaataccccaagctccagccccaccgaacttctcaacattccacacaatgccttttcactactctgtgtctttgcatgagttgtttgctcttcctagaaatgctctcccgccttccctcacctggaaaacttctactcatttaagattcagcttaaaagttgcctcttctattaagacttattttcccagtcaaaattagtcactccctcttctaggatctcatagtcctatctctaataaattatttattatttgttttacatttctttatatccccacctgactcctttacagcagtaatatatattgttcaaacatacacccttaaagtctataagagaaagtctgcaataaatgtttgttgagtgaatgtccccatcgctgtggttaaattgtatatgcaccaccagaagttgaacagactccaaaactgaattcagatggcttctgtgaatgaagttactctagataaaggggtaagggatgacaaccatcattcattcatagaaataacacaaactcaaaactacatttgagggtcacccaaaatatattaatagtcatgatgactcacatataatgtcaggaagaaaaatctgaattatgacttttataataatgcttatttggctttttcttatgataaaatttatatataattattatgataaaattaaagtagatatgtagataaataaaaacagaaaaaatcactcataattaaaccatccaggcaaaattaccattaacattttggtgtacctcttttcacacatacaaaaatttgtatgtgctttatcacataacaatatatcgtgagtattttccatttaattacattttattctaaaccatgactatatatcagcccgttttgtgtgtgcatatacaataatgaatttatctacttctattcttggacataaaggttgcttccaacttttcagtattgttaatagtgccaaaaattatccctgtagctaccaatacttcatatcaaaagattgtgctaatttcccagtaacaagtcaagtatgagtgcctgtttatctaaaactcttgctaactatgagcatttaggctgtgatctttaactagaaaagagcaaatctaatcaactatacggtattttgtatctaataaaaataattattttcagaatggggatgggggataaggcacctgtaaacaggatggtcaaagataaaatctggtgatgcatctgagcccatgaacacgagtattctgtttgtacagcaggaaccttctgaggaagatgaatgcctcagggtcaccatgtttgatggtcctgcctctcatgatcatccactttctccacctttggtctctgctcacctggctacatgcagcctcggggaaaagcataaccttctaccaacaagagcccgatggtcttgttaggctaacaacaaggtagttctcactgtcagttgtcactctaatccatgtatcagtcacatgtcataattgtgttaatgtgagtccatctccagaagacttattacctctggcaaggaattttctggaccaaaattagaggtaaaaccttagatcgtttccaaacttgctgcccaacagtatcactcaaccaaggatattttgttttttcattatttttttttaatgttgacttccaagacctgtccctggagattctaatttgggaggtatgggataagacctaggaatctctattttttaaagctccacagctgattctgatgtaagccaaagactgagaactatggacctagactgtgatggcctaaccagggtccttatccttcaaagctggtctaagagagtagccagctttctctaagtaatagcttttgtttctctctatgccattctcaaatagcaacaggttaaacctaggataataacgcctaacgtgtcttgttcttactgtgttcctcacaatatttctgagtcctaaggctcagtttcctcatctgtaaaatgcagtaacaacctacatgtcaatacttatgaaacaaaataactactatgacaagaaatattattttagtcagagctttccttttcatcacaactctaagcctggctctaagcctgaaacacaacatagacagaaagtagtagtagtaagtgaacttttttttcagtgggccaaactcaaatgttgaatttgcaaagcagttgtatgagctgtagcaacttttggaaaatgtcgtctaaaactcttgttgaaaatggagaaaatctcacctctccaggaccttttcctttactctgctttgtccctgtaggtctcctagggattctgcaaaagctgctgtggctgtaactccccgctggcttctctaatggcgagagtatggcaacctctctgagggtgggacttggttggagaatctccaaaccgggccaaagccagctgggctctgctgaaaatgaggaaagcccagtcaaggcctaatacccagctaccactccaactccaagcccaagtgctcacagcacccgaaatgaagagaaaattcaaaacaaattcctgcattttgtcctaatcagaataggagtccttatgcccttgaaaagatgaggagttcagagagaaaagggggtgctagacagcaattcggcaagtagagaaaagcaatgcatatgactttagttctacagagtggacctatcttcgatctactttgttattgtaactcaaataacaaaaagatggtctgatcatcttatgatggccatcattaggccttgtgttgggacccactgctcttgcctatacgatggcaagatcttctttcacattagggtggaaccaggaccacttcatacattctaaaaggcaggcagaggatcctagggaccaacccagtgcatacccatatgccaaacaaaccagagcacccaaaggctcgagatggggagaaccaacctaccatcctgcacaacatgctcatccccaggaccagaccaggactggagcaggcctgccacctgatctccttcagctttgctcttacctcaggcctcactctgaaaggtcttagcagcaaaggagtttctaagactaagagctgggcactggaaggcccagcacaagttcatggaaaatacaactcaagcctgagggagaagccctgcctgcagagaacacagttatgctgcatctcacaactacccaccaagtactggccctcctataatgatcccatagcagtgggtatcagaaggctgccttttcttagggtcctgggttcctcctttgtcttcccacatcagccccaggaagcctgggaatgcatggggattagagtagagtctgaagaaggagaagggtggggaaccaatactcagctggggagagacgaacttttacaggtgagcaaaaaattgtctgtgaaatatctgctctcagtgggccaaggtgagcatattgctgagctctgtctgtgactaaggatggctggaaacataaaatgcagataattttgagtttgtttttctatttcaataaagaaaaatatatatttggactttttttctccctctttctggatgtagcattagctggcttcctccacaataagcccccaaatagaacacatgcgtgagaggtgggagcattgaggacagcccaaagacaaaattagaaccaagtcctgggagacagcagtatcctagacttttcacaaaatctgctttccaaatccggctccaataacactgctcttttgcaaaactggcaacggttgccactgagaatctcaacagtatatcatacttgtcaatctgggttccttggcaatgattcaacctgttgtgaacccggtatttgcttctctcctcacccccacattagctatctcccctagatctctttgatttcttgtttacttctctcttctctgtttgtctcattgttaggaggccacagccaaataacgggaaaagaaggcaaggcagatgctgcttttattttgtagctattgattatacgaaacacaccatctctgggaaaaaaatggggctaaataactgaaataggcaatttgtagagactaaccctgtgtgggcagggatacattagttgagctctagtgtgctcagatctcatttctgtgctcagtgattctcttcatctggtttgctgataagtgaatctcatctttcaagacaggctataagtgtcaaattatttttctcttcttctcctgataggatacttatcagcagccagcatcctgtaagtgaaggtgacctcagatgggatgaaaagttttccctgtcagttccagccctgtagatggatcttcatcccaggtggaactgggtgcgaatgaacttgtttagctcagcaaatccaggaaactcagcaggcaggaatgctgcattgatcttgtcaagtgcagactccacatgcagaggttgaggaaggcagtggagacatgcactctccagcaggtggccacctccttgacttctccatcttttggcatccatcacactgaactgccttgcttctcctcagtagcaattattcctcttcagtcttcttcaaggctcctctcagctgcctttcccctccatgtcctgtctcccaggctcagcccttagtccttcttacttctcctataatttcttctcaggccatcatatacattcccatagtttaactctatttgccactaactcccaaatccatatctctattcttagcctctctcgctttagctcctccatttccaacaatctgccagtcattgccaccaggatgactcactggaacttcccatccagactgtccaagtaaagcattttctttctccagtgatttggccctttcttctgacttccctatctctagcagataccatcatgcagatagtcacccaggcaaaacaaacaaacaaatgaacaaaagttgtcgtctttcatccctccatcttcctcacttactgtagtctactagttttaaaatataaaaagattctactcctgttcagaaagccttcagtggccttccattatctgttgat

SEQ ID NO: 14009 - RNA, 2150 nt, Homo sapiens
  source 1..2150: mol_type = other RNA
gctgggattacaggcatgagccaccgcacccagccgggacaaagcagtttgaatgaaggataatccatgtagatagtgaaagagagagaacaatggcttggaaatgagaagacagaagtcaactggattggcaagattggaaaatctaggctgtggaaaatgagctagaggcaaagttctgccgtcaagagaacccctagaacaatgatatgccacttgctgtaggcaaaggtggccctcctccccagcctcagcctgggggacccactaagccctgtggggcaatattctcctttgagctcttcaaaaggtggtcactgtctcttctgccccagagtggctgccatctagggtcgcaagatcatatttccaacaccagtgagaagtgagaagatacagagaaacaccaggattgactactacctcatgtaatccttacagtttaacttgtgtacagttagacacttctgataaatgaggaaatggagggtcaggtaggttaaaagtaacaggcccaaggtcacacagctggtcaatggaagaggcagatatgagccaagatttctcctctactccaccatgccttctaccttatgggatttgaagaattctcacacaaatcactgtttaaagccaagtcattcccacctctggaaggcagaattaatgcccttatggctgcaggtcactcaacagttaagcataagctcctggccatgcagatgcccagagacttcttgcagctctgttccagagaaaccaagagctgcctctgctttcctagtgtgtctgtggactgaccaagcttaatggctggcagtcacgttgtcaacacagacaaatacagcagggctcaagcaggagggcctcctgccaggcacatgcaaaatgcatgctctgcagggcagagggtcagagcagctaaaagacagagcaaccagggattctgttccaggacctggtttcatggcaccttctcaatttatcaagctgaaacaccaagtatcagcatctcctgatgagaaatcctaagacaggatccgatttcccaccttgtctccatctctcacatatgccaatctattttaaactcccacaaggaagtggggactttccgaggcaggtaacccctatccaagggtcatgccttagagggataagccactacaacagaagagagggcactgcacccactccctttaccccttcaaaaggggcaggctgctcctaaaaggtaggatctcaacctgctctgttacataacttccaaacttcctgcggaaatatcaatcccattcttcttgttttaccctctgaaaaaatcctctttgcagatacctgtatgcaaagttcctccagccttcccttctcccaacttagtcagcccaacttctttagggctctttctcagaccctcatgtgcatggctccaattccggattttcttccactttttaacactgctcaggcacaaatgttgacgtgcttcctcaagggacctaacaggtgacgcagaattagtgagcactttgtcctgaagtaatcaagtgaaatgttagaggcagagctctcactattgaccctaccaatggaaagggacaaataggcccaggggcatatgcctcctcctctccacctctactctccttgtaccagaaaattcacatgggactgactattcactaggttctgggataagattctggctcgagagaaggtagtgtcacctagaaggcaaggtcatacaacggaaagaacaccagcaatcaggagatccatgttgagtttcacttccattactcagtagtgtaagactggaaccaagtcacttcactgaaattcagtttccttgtctgttgaatcgggctaataaagcctatcaatgctgtatatgatatgcaacccccagactatccgtcgttcccagcgaatgccgtccgctggtcgcatcttcctccatatccactcggctcccggtactgccgcaaccggaaatttggactctgttattaacgcccccttctcagactccggcggctccaccgcgtctgaggcgaactccaagcccggacctctaggccgcagcccccagtctatccgtcgttcccagcgaatgccgtctgccggtcgcatcttcctccatctcgact

SEQ ID NO: 14010 - RNA, 95 nt, Homo sapiens
  source 1..95: mol_type = other RNA
gctgggattacaggcatgagccaccgcacccagcctaaacttattttcattactgttaagccaaacataatcacagcataatcccagctaaaatt

SEQ ID NO: 14011 - RNA, 3687 nt, Homo sapiens
  source 1..3687: mol_type = other RNA
gctgggattacaggcatgagccaccgcacccagcctatacacacatatttctaagacaagacacttactgagataacatgactatcaaaacccattaactgggcaataaaccatacagacagttcttaaaaagatagaaggttttgtgtatgaaaactgcacctcaatgttttaagataaatggttccacacaaaaatatgcatctacctctccttttggaaaaccagactataggataacacaagatttacttattattaaggattcatctcctcacaagttaggaaggacagccttctcagcagtggcaataaacgggaagtaataaagataattcctaactggcacaacagatctgggtgaatcacaaaaaccacatatctggaaggcaaggtgtatgttctctcaaatcctgctttcctgcccgtgcagcaatcatctcaaaaacagtacataagttatgagtccacaaaatctttagatgccttatgctgacgatgtgtgttgctaaaggagaatcaaaggtctgaggtcctgagaatttctatatacccccaaaccatgaagccatagtaacacagacatatctggatgcacctttggatgggacacattcactcttcttggccacaatcttttctactctgtttatcacacctacctgtctgggccaattactgttcttacctggccccagtaggtcttacaaccagtgacctacctaccaattcagtccttcagtgcccatggctacaatgaaggacctgggaaataagataccatgaacagtgctgggaaatatgaagcatcactgcaaataaacaattcatgcaggtcccagcacttgagtttgtcacaaatgcctcttctcagggagacctctggacctacaaataaatctggcatcgacaccatgattaggaccacacagctctgctctccttcctaggagaccttggaaaccaataaaaattaagacaaacaggactaagaactattttccgatctcatactatgtccctggggggacataaagttggagctgttcacccttcacactggcagagcacatacatcagcacatggtaagacagcccatttccctcttgggtaatgtgggagagggaatatcccactatggcaatcacataaaaaaaaaaaaaacctatgaagaaggtaaacctccatgggctacaagaatccagattgctcttcttggtcaaagttgggttttgtctttgcctcgaacagttcagcaagatggaagaggaccctcaacaggcttttattatattattcccttcagaatttggtaagcacagtggtctgcattccttgagcacatgtgagtgactgatgaaaacggtgaggatatgccacatggtagtgtctgttgtaacactgggcagattagaaagtacaagtaatctctagaaagcttcccaagtacttggaccttgtagtgaatctttcaactagtgatatgcagatgtatgagggtgaatttctgtctgttggatcccttgaaaaatcagctctctggtgtcctacagtgaataagacaattacacatcccaacaattgctagggctcttctgttatatgtaccttctggtgcctgacaagggaatatcttttgttgaaggctttcccacatttaccacattcatacggcttttctccggtgtggattcgctgatgctcaacaagtttgtttttatagataaaggccttctcacatgcagtgcagttataaggcctctctccactgtgaactttctggtgttgaatgaggctggtgcggtgtctaaagcatttcccacattcactgcactcacagggcttttcgccagtgtgaactttctggtgctcaagaagtcttttttggtggctgaagacttttccacattcattgcactcacaaagttgttctctagtatggattctttggtgctgaagaagtttaacctcaaggtagaagccttttccacattcactgcattcataaggcctttctctagtgtggattttgtgatgcttaagaagtgtttgtttggagatgaaggctttcccacagtcactgcattcataagccctttctccagtgtgaattctctggtgtcgcatgtagtcagacgagcggataaatgatttcccacatatgatgcacacataaggcttttctccagtatgaattctctggtgctcaagaagtctttttttgtgaatgaaggccttcccacattctttgcactcataaggcctttctcccgtgtggattctatggtgatcaagaagtgactgtttgtatatgaaggatttcccacattcactgcactgataagccccttctccagtgtgaactctctggtgtcgaatgcggtcataggaatgaataaaagatttcccacattccatacacacataaggcctctctccagtgtggattctctgctgatggccaacaaatgtttgtttgtggcggaatgatttcccacatacattgcacacataaggcttttctccattatgggttctctggtgttccacaagtgagtatttggagctcaaggatttcccacattcgatgcacacataagacctttctctagtgtgaattctctgctggtgcccaacgagtgtttgtttatggaggaatgatttcccacatatattgcacacataaggcttttctgcattatgggttctctggtgttcaacaaataagtatttagagttcaaggatttcccatattccctacgcttataagctttttctccagtgtggactctctgatgctcagtaacatgaactttctcattgaaaacttgctcacatttgtaacgtctttgttgaaaggtctccctgcttctatgtgcatactcttgtctgctgtgggtggtctggtgttggagaaggcccaggatggttggaaaatccttctcaacatctttgcatgggaaaagattgtctgacagaggaattttgcagctattcagaagcaaggcactgctctcctcctttctgatgtgtttctctccactgtcctggttctggtgctgttgcaggttagaaccaaatgaaaaccatttcccactggccacagacgtataaggtttctgccagggaagtgtcccctgatgctcactgaggtacaaaatgtctttcatgaccaggatacacatctcacaagaatgagcatttgggatggaaggacctagctttggagtcctggcctgtgacactccttgcgcagaaagagtctgctcagaaggggcctcctcagcctctattccatgcaaacaacctactgaggccataagcgaaaagttctccagcatcacatcatgatacaggcacctttgagcttcatcaaggaggccccactcctcctgggagaagtacacagcaatatcctcaaaggtcacatggccctgcggcgtaatcactagcgctgcctcggccatgggactttaggcggggcggggcctggaaaggcgggcggtaaagcccgggatccggcgtgcgtgcggtggcaaatcgctgggcgacgctcagaccgagaccaggcaagctcctctgcgggcggacaccacctccaccggtttccggctccagttacctggcccggacccagcgagccggaaacgcccagcccgcggacgcgctcgcaggcagcaaaaac

SEQ ID NO: 14012 - RNA, 3726 nt, Homo sapiens
  source 1..3726: mol_type = other RNA
gctgggattacaggcatgagccaccgcacccagcctatacacacatatttctaagacaagacacttactgagataacatgactatcaaaacccattaactgggcaataaaccatacagacagttcttaaaaagatagaaggttttgtgtatgaaaactgcacctcaatgttttaagataaatggttccacacaaaaatatgcatctacctctccttttggaaaaccagactataggataacacaagatttacttattattaaggattcatctcctcacaagttaggaaggacagccttctcagcagtggcaataaacgggaagtaataaagataattcctaactggcacaacagatctgggtgaatcacaaaaaccacatatctggaaggcaaggtgtatgttctctcaaatcctgctttcctgcccgtgcagcaatcatctcaaaaacagtacataagttatgagtccacaaaatctttagatgccttatgctgacgatgtgtgttgctaaaggagaatcaaaggtctgaggtcctgagaatttctatatacccccaaaccatgaagccatagtaacacagacatatctggatgcacctttggatgggacacattcactcttcttggccacaatcttttctactctgtttatcacacctacctgtctgggccaattactgttcttacctggccccagtaggtcttacaaccagtgacctacctaccaattcagtccttcagtgcccatggctacaatgaaggacctgggaaataagataccatgaacagtgctgggaaatatgaagcatcactgcaaataaacaattcatgcaggtcccagcacttgagtttgtcacaaatgcctcttctcagggagacctctggacctacaaataaatctggcatcgacaccatgattaggaccacacagctctgctctccttcctaggagaccttggaaaccaataaaaattaagacaaacaggactaagaactattttccgatctcatactatgtccctggggggacataaagttggagctgttcacccttcacactggcagagcacatacatcagcacatggtaagacagcccatttccctcttgggtaatgtgggagagggaatatcccactatggcaatcacataaaaaaaaaaaaaacctatgaagaaggtaaacctccatgggctacaagaatccagattgctcttcttggtcaaagttgggttttgtctttgcctcgaacagttcagcaagatggaagaggaccctcaacaggcttttattatattattcccttcagaatttggtaagcacagtggtctgcattccttgagcacatgtgagtgactgatgaaaacggtgaggatatgccacatggtagtgtctgttgtaacactgggcagattagaaagtacaagtaatctctagaaagcttcccaagtacttggaccttgtagtgaatctttcaactagtgatatgcagatgtatgagggtgaatttctgtctgttggatcccttgaaaaatcagctctctggtgtcctacagtgaataagacaattacacatcccaacaattgctagggctcttctgttatatgtaccttctggtgcctgacaagggaatatcttttgttgaaggctttcccacatttaccacattcatacggcttttctccggtgtggattcgctgatgctcaacaagtttgtttttatagataaaggccttctcacatgcagtgcagttataaggcctctctccactgtgaactttctggtgttgaatgaggctggtgcggtgtctaaagcatttcccacattcactgcactcacagggcttttcgccagtgtgaactttctggtgctcaagaagtcttttttggtggctgaagacttttccacattcattgcactcacaaagttgttctctagtatggattctttggtgctgaagaagtttaacctcaaggtagaagccttttccacattcactgcattcataaggcctttctctagtgtggattttgtgatgcttaagaagtgtttgtttggagatgaaggctttcccacagtcactgcattcataagccctttctccagtgtgaattctctggtgtcgcatgtagtcagacgagcggataaatgatttcccacatatgatgcacacataaggcttttctccagtatgaattctctggtgctcaagaagtctttttttgtgaatgaaggccttcccacattctttgcactcataaggcctttctcccgtgtggattctatggtgatcaagaagtgactgtttgtatatgaaggatttcccacattcactgcactgataagccccttctccagtgtgaactctctggtgtcgaatgcggtcataggaatgaataaaagatttcccacattccatacacacataaggcctctctccagtgtggattctctgctgatggccaacaaatgtttgtttgtggcggaatgatttcccacatacattgcacacataaggcttttctccattatgggttctctggtgttccacaagtgagtatttggagctcaaggatttcccacattcgatgcacacataagacctttctctagtgtgaattctctgctggtgcccaacgagtgtttgtttatggaggaatgatttcccacatatattgcacacataaggcttttctgcattatgggttctctggtgttcaacaaataagtatttagagttcaaggatttcccatattccctacgcttataagctttttctccagtgtggactctctgatgctcagtaacatgaactttctcattgaaaacttgctcacatttgtaacgtctttgttgaaaggtctccctgcttctatgtgcatactcttgtctgctgtgggtggtctggtgttggagaaggcccaggatggttggaaaatccttctcaacatctttgcatgggaaaagattgtctgacagaggaattttgcagctattcagaagcaaggcactgctctcctcctttctgatgtgtttctctccactgtcctggttctggtgctgttgcaggttagaaccaaatgaaaaccatttcccactggccacagacgtataaggtttctgccagggaagtgtcccctgatgctcactgaggtacaaaatgtctttcatgaccaggatacacatctcacaagaatgagcatttgggatggaaggacctagctttggagtcctggcctgtgacactccttgcgcagaaagagtctgctcagaaggggcctcctcagcctctattccatgcaaacaacctactgaggccataagcgaaaagttctccagcatcacatcatgatacaggcacctttgagcttcatcaaggaggccccactcctcctgggagaagtacacagcaatatcctcaaaggtcacatggccctgtgatggtttcacaaactcttctgttaccatgggaatctgcggcgtaatcactagcgctgcctcggccatgggactttaggcggggcggggcctggaaaggcgggcggtaaagcccgggatccggcgtgcgtgcggtggcaaatcgctgggcgacgctcagaccgagaccaggcaagctcctctgcgggcggacaccacctccaccggtttccggctccagttacctggcccggacccagcgagccggaaacgcccagcccgcggacgcgctcgcaggcagcaaaaac

SEQ ID NO: 14013 - RNA, 2200 nt, Homo sapiens
  source 1..2200: mol_type = other RNA
gctgggattacaggcatgagccaccgcacccagcctatattacatctttaaaggggttgaacaaaatgcccaacaatattataaataaattagaacaagaagtccatgctgctgaatgacatggttgaaatgtctgttcaatatctctgattctacattcttgaaactgtttttttttaaaaagaaggtgatgtgaacagtaattttccttgcagcaaacccagctaagtaataatttctagcacacctcgaatttctagcaagagtgcaatgtggtcatttagtcacgcatgttgccagtcactctgagcccacagtgcacataaacggtggcttgcatctcattgcaatcttggcttcttggcctgcaaaaggtggtcccagcaatgcagagatgccattagcacagatgatgatgccgtaggcattggccaggtgttcaatgccaaccaagtcttcagtcactacgggcattagggagaaataaccactggaaaaccctatcagcgcacagatgaccgccaggccagcgtacgtgtgcatcaacggcagaataaaaatactgaggacaagggtgaagttggccaacaggaagacattccaaacactaatgcaaggcaagtcggctatgacgcccaggatcacttttccaaagatgtgaactattgctataattgacgtcagagggaaaacgtcgttttgctccgataagttatacaaattgacgatttctgggaggtgaatgaaggggatgacaaagctgctgtatgcaaacaaagcccagaaaataaaggctacaaacattcgatttgtaaatagagaggctgtcccaaagtagcccgaataccagtcctcgaagcccttcctgactctcatggtgagccagctgacagtcttcagaatccggagggcacacatgttcttcctgtgcccggcctgatcggggcactcctgggcttgcaggtcgcagagggtctcctcgttcccgagcccaccatccttctcttctgttcttccctgctgtccagttgacttcacagattctgtggagtgcgctggcaggccacgcacatctttctctcctgggtcgtttgggtttttaccaggagagaggggcctcatgagcgccccacaaacacacaggtttagggaaacggcaccttggatcaacatggcattcctccagccgtactctgcgcacaggtacttcagcagcacagtcattaggaacgtaccgaatccggtccccgtggtgctgaggccctgggcgagggcgcgtctcttctggaaatacctgcccaccatgaccaccgctggcaggtaggccatcccgctgcccaggccagctgcgactccaaaagtaatgaagagataatgcacgtttgcagcataggcactcaacacccagcccagggagttgacgagccctccaatgatcgcagtctggcggcacccacaggtgttaatgaacaagccgatgaaagggcccactatcaaggtgatgcccatgctgagggagctgacccaggcggtcaggccgcggctctggtggaattcttccagccattccacgttgaggacacccagggccatctgggagcccatgatgaggatgtgcacaaagaaagaggagagcaccatcatccaagcccatccgccatcaatgtttgggtggggcttcagtgtctttttgtctttggggccatcttcaaaatcatacccaatatcttcatgactggtatacattttccaagatttttcgcccgaggcccgctgggctgcggcctcactcggctccacgcccggatcctcgaacttgctgctctgcttggagccccctgagctgctgggtgtagagatttgttgcaatgtcgcctatcatcctggagacgcgggtgcctgcggctcagctctccgcccggctcggtgcgctctgtgaggggctcccgggctcttccgccgctcgctgccaggccaggtgagcgtttggtggagctgaaagctcgacgcctcagtccaggtggctttaaaacgggtgcgtttggaggtgcccaaacctaacctgggcttccttccaatcggagcaatttcaaatcttcatgctcgttcattcctataccggctaattctggtttggcagggaaaaaaaatgcagtcacctcacatgcacactcttgtggccggttgaagtttatagctt

SEQ ID NO: 14014 - RNA, 1418 nt, Homo sapiens
  source 1..1418: mol_type = other RNA
gctgggattacaggcatgagccaccgcacccagcctatatttttttatttttttgagacagggtcttgctccatcacccaggctagagtgcagtggcccgaacatggctcactgtagcctcaacctcctggacccaagcaatcttcctatcttagcctcccaagtagctgggaccacaggtgtgtgccaccacatctgctaatttttctttttataaagacgggatctccctgtgttgcccaggctggtctccaactcctgggctcaagtgatcctcctgtcttggcctcccaaagtgctgcaattagaggtatgagccacagtgcctggactattagtgactttaaaaggttccattcatcaggcctggtgcagtggcttatggttgtaatcccagcactttgggagactgaggtggaaggatagcttgaagctaggagttcaggaccagcctggcaacaaagcaagaccatgtctgtacaaaaaattaaaaaattagctgggtatggtggtatatgcatgcagtcctagctactctggaggctgcgagggtaagatttctagagctcaggagttcgacggtgcagtgagctatgatggtgtcattgtattccagcctaagcgatgaaatccaaaggtgaatcttttggttggtgattttgatgatagccacaaagcaagcagggtgagtatgatggcgcttaggtcagttaacatatgaagtgcatctgtcatgattgctaggctatttgcaatgtatccacctacaagttctccaatcatgaaaagcaagtacagaacggcagcaatggtcaacctggctttcacctttctctgcttcagtatctctctctgtttgctgcagttgtcacaggagtccaccttcaaactcagctgactgttggtcaaaggtaagtcttggtccagtaaggaatcatcgtcggcctggagggtcgggtgcgccccgttaacaggcctttccggggcttcggaaccgtcatcggccaccacaactcgaagtttgttgaaccgagaaagcccctcgtcccccgcctcatccgagaagtcaaaggcgctggtgtcatttaaaaacagcggcgcatcatccttccttagcatagatttgaggcgcttccacgcgccagagccggccatggcagaggctgagcggccgcggtgcggaacggcttgggggaggcggacggccggcggcgcctacttcaccggagcgccagttctcgagggcagtgccgcgcgtccctccccatcctggggcgctgccgcggggccgcaactcatctccccgcccccggccggctcagcgaggcgggctcgcgctgctccacccgcggccgcaggagagtggggtcgtgctcgcgcccgccgcgcccgctgctggaggccggctccccaggtct

SEQ ID NO: 14015 - RNA, 1695 nt, Homo sapiens
  source 1..1695: mol_type = other RNA
gctgggattacaggcatgagccaccgcacccagcctatgttggctatttttgtcattttaagcaatatattccttctatttgtgtgcgtgtgtgtgttgttccataagcctctgtcaacgtcttttgcctcccttgctccatataaaatgccttacattcctccctcttttcccctacccttattcatggaataactgtgaatcattgttaggactttattgttatgaaagccaataatcttttatcttttattctacaactacaattaagtcttacatgtctgtaggttgattctaaaagtagaaaactagagcagcctttatgattttgtctacattgctcaatgtagagccagggctgtgccaggatgccatttccttccctccatgtcctgtgcatctgtcatggtgctcctggggcgatgctactcacttcatagttaagcaggctcccttcccacatccttcatcaaatgctccatgtcacagtaaaataagggtcacacgtgagccatttctttataccttgttttagatgatttttcctctagttttagatgatttttttatccttcctattggaaaaggataaaaaatcttaggaacttccattgtgtcctaaaatttatctgccttccaatcacactaccatgtgaagtccttcttccccagagtccttaattgttctgaatttaagtggattttctctgggctgaatgcacaagccttcagcctgagtcttctgttcactgggttcctggagccagtgctaatctccaaaatgtgtcctttcttggtttccatcttctttgactggagtataacctccagtaaactcctattaaatctctactgttgccagtctgcgctcctggattttcaaggggctccgtggaattgggaggctgatgaagctggtgaccaccctccgtaagcatgctgtgttggtgattccagtgcttactcctttcctcaaatgtggtcataagaagtcaggaaagtcaatatgctttcaatcatcctgtggtctgtatgctctgtggctacacacctggctgagaacagaattaatgatgagaaacgtgcctgcttctctgcataaaagatgatgtctgagtagaaggtcgccaagggaggattaagagcaagaatgcgagaatgtgctcaggaatccgtgcgtgagatgatgagcttgtgagctgatgttgattctgtgcagttcccagtgtcttattcacaggcaagattttcttgctcatcgttcagccttcaatgttttaagcaaagatttttaaaaagatctaacaggaaacgaggagctgcagtgaagcttgggcagtcagttcgaatctgaataaatatttgtcagattggagaagcgctgaaagcattaagatacttggagatttctctttttctttggcaagaagcatgactgagacaggtaagggctaggaattcttccggatcactccctccaacaatggtctttcctttgaatttgcactttggagtctgacacagattagtgcttcctagtcctctaactgtaacacatgcctcagtttcccttctccgataagattgcaatatctttgggtgcaggaaaaaaaatagttgatccttttctttgtagcccagcaagttccaggcacattagaaactgattagaaactggtacacaagtgttacttg

SEQ ID NO: 14016 - RNA, 1044 nt, Homo sapiens
  source 1..1044: mol_type = other RNA
gctgggattacaggcatgagccaccgcacccagcctcattctagcatttatatctcatcgttttgtgatgtgggcgagattatctgtctccttttagtgggtgaaggcctccggagttggcatcttatccacagctctgaacacagcaccctgtttcatgtataaagtatttactgaatgagcaaacaaatagataaagaatagttgcccctgttagatggtatctgctcttaccaccacttcagccccgccccaggcactgaccccatcttccctgccaaggttaccagtggcctgtgaatacatctcccagaatttgaccctcttacacatgttgactcttactagccaccattctttatgttcttgacaatgtgcgcttctggtctttctcttccttctctgaccagctcttcttggtccctttggggcgcagctctccctggtcctctggggttccgttccagtccctcttttcttctcaccatttacccctcttcctgggagagtgcattggttctctctgctgctgactcacaagtctgtttctctagctggaaacttcttggtcatttcaacctgcatgttcaaggaatgacctttgtctccccacatctcccacatctttcctcgcagcccatcatcaaccaggcctcagatctgtccacttcttgccatccctgttgacagctctgggtccatttcccacctggatcactgcagcagcctccttaaccagcttctctaagcctagtctttctgtctcattcccttcttcacccagcatatgaagtccaaaaatggatgtattggcaggtggctcttctccaagtgcttattcagagctcctggtcccttgcatcttgtggctgtgccatcttccacacatggcctctgggggtgccaagctcatctggcatttgaatattgattgagattctgctggcctctggttcgtgctcaggaaaacccccctctcgttatagcccagcttcgttttgctgagatgtctttcaatgtttccagcagcggtgggggtgggag

SEQ ID NO: 14017 - RNA, 1383 nt, Homo sapiens
  source 1..1383: mol_type = other RNA
gctgggattacaggcatgagccaccgcacccagctatttttttattattattattattattttaaagacaggttctcactctgttgtccaggctggagtgcagtggtgtgatcctagctctctgcagccttgaactcctgagctcaagcgagcttcctgcctcagcctcccaagcagctgggacaacaggcatgtgccaccgcccctggcaaatttttaaatttttagtacagatgagatcttgctttgttgtctaggctagtttcaaactcctggcctcgaggtatcttcctgccttgaccacccaaagtgctgagattacaggtgtgaggcaccacaccctgcgggtgcacactccattgctgctgtgtctgctctgctcctgcccccatgcttcagataactctgccttctgccagacccacccccatcctgttagaacccctggaaggggcagcaggcatgggggacactggagacatgggcgtgctctgtgtgggctgccacctggagcagggtcccttggccacaagtgctgggatgctctgttggttcttgctgaccctgatgctggtgctgggcctgggtagggggccttgctgccagatgcctgagtagggtgtgagtcatggccctggccacatcaggggtccctgaagccacaagccccaacacatcagcctctgtgtcatccaggctgccacggaggatgagggggcaggcccaggcactagtggtagacttggccaccaggttgctgagcagaaccccagtgcttggggacaggtgtgcagagccaaaggagcagttgagcgaggaggtgagaaggagcacagagccgctgctgtccacggcggccagggcactgctctcggggctcacagcagtctagccccgtggcatgaggatgcaccactgccaggcacaatgcagctccaactccagcatccacgacgttgcccccggcaacaagcagctctcggcctgcagggctgatgatggcaccgtggtggtatacgccagggccgtgggagtgtccgccgggtggaggggccacagagcccaagcttcctgtcgacctgccctgattctggagctgcctcacagccagggagcagccaacagccagcagcagcagggctgccactacacgggcccaggttccgggcagcccgccagccttgttcctggaagagtcctggtgcctccgggggtttagaaccagcgcctctgatgtctcctcctcctccacttcctcctccgactccaagcttggctcccagggcagcagcttctgatagaccacgggctcttctgcccgctccatggccccccagtgctcgccccagccctcctgcctgccagcctttccggctgtgtctc

SEQ ID NO: 14018 - RNA, 1991 nt, Homo sapiens
  source 1..1991: mol_type = other RNA
gctgggattacaggcatgagccaccgcacccagctatttttttattattattattattattttaaagacaggttctcactctgttgtccaggctggagtgcagtggtgtgatcctagctctctgcagccttgaactcctgagctcaagcgagcttcctgcctcagcctcccaagcagctgggacaacaggcatgtgccaccgcccctggcaaatttttaaatttttagtacagatgagatcttgctttgttgtctaggctagtttcaaactcctggcctcgaggtatcttcctgccttgaccacccaaagtgctgagattacaggtgtgaggcaccacaccctgcgggtgcacactccattgctgctgtgtctgctctgctcctgcccccatgcttcagataactctgccttctgccagacccacccccatcctgttagaacccctggaaggggcagcaggcatgggggacactggagacatgggcgtgctctgtgtgggctgccacctggagcagggtcccttggccacaagtgctgggatgctctgttggttcttgctgaccctgatgctggtgctgggcctgggtagggggccttgctgccagatgcctgagtagggtgtgagtcatggccctggccacatcaggggtccctgaagccacaagccccaacacatcagcctctgtgtcatccaggctgccacggaggatgagggggcaggcccaggcactagtggtagacttggccaccaggttgctgagcagaaccccagtgcttggggacaggtgtgcagagccaaaggagcagttgagcgaggaggtgagaaggagcacagagccgctgctgtccacggcggccagggcactgctctcggggctcacagcagtctgcaggaacggtgggcaggggtcagggatgggcgccccggagcgcagggctgcctccaacagtgccagcagttctgggccagctgagggactgggggtggtgaacaggatgccctggggcacaggtagctgctctgctggttccaaagtgggcctgggcacagccgagggcacctccacccccaggtctcccgccagtagactcagtagagcatccccagcaaggtctgaggtgggagcgagggctgcgctgcgaagcacagctgccagttgtgggttggtggctcgggccccagcgcccaggggtgtcccatcagcatggcaaagtagtggacagaggccttctgtgccccgagccaccagagcccttgccaggggtgtgtccaccaggaagccctcctgagccagcgtggtggggcccactagcaggcgtggccagggcaggcggccgaagcgtgcatgcagcaggtgcagggtgggcagagccgcgggcagccccaggccgggggccagggtctgtgctgggcctgatgtcagggccgtggaattgcctgaggagctatcgtggaagaggccccaaaacatggcacctagccccgtggcatgaggatgcaccactgccaggcacaatgcagctccaactccagcatccacgacgttgcccccggcaacaagcagctctcggcctaggtgggagcatgtggctgcagggctgatgatggcaccgtggtggtatacgccagggccgtgggagtgtccgccgggtggaggggccacagagcccaagcttcctgtcgacctgccctgattctggagctgcctcacagccagggagcagccaacagccagcagcagcagggctgccactacacgggcccaggttccgggcagcccgccagccttgttcctggaagagtcctggtgcctccgggggtttagaaccagcgcctctgatgtctcctcctcctccacttcctcctccgactccaagcttggctcccagggcagcagcttctgatagaccacgggctcttctgcccgctccatggccccccagtgctcgccccagccctcctgcctgccagcctttccggctgtgtctc

SEQ ID NO: 14019 - RNA, 1973 nt, Homo sapiens
  source 1..1973: mol_type = other RNA
gctgggattacaggcatgagccaccgcacccagctatttttttattattattattattattttaaagacaggttctcactctgttgtccaggctggagtgcagtggtgtgatcctagctctctgcagccttgaactcctgagctcaagcgagcttcctgcctcagcctcccaagcagctgggacaacaggcatgtgccaccgcccctggcaaatttttaaatttttagtacagatgagatcttgctttgttgtctaggctagtttcaaactcctggcctcgaggtatcttcctgccttgaccacccaaagtgctgagattacaggtgtgaggcaccacaccctgcgggtgcacactccattgctgctgtgtctgctctgctcctgcccccatgcttcagataactctgccttctgccagacccacccccatcctgttagaacccctggaaggggcagcaggcatgggggacactggagacatgggcgtgctctgtgtgggctgccacctggagcagggtcccttggccacaagtgctgggatgctctgttggttcttgctgaccctgatgctggtgctgggcctgggtagggggccttgctgccagatgcctgagtagggtgtgagtcatggccctggccacatcaggggtccctgaagccacaagccccaacacatcagcctctgtgtcatccaggctgccacggaggatgagggggcaggcccaggcactagtggtagacttggccaccaggttgctgagcagaaccccagtgcttggggacaggtgtgcagagccaaaggagcagttgagcgaggaggtgagaaggagcacagagccgctgctgtccacggcggccagggcactgctctcggggctcacagcagtctgcaggaacggtgggcaggggtcagggatgggcgccccggagcgcagggctgcctccaacagtgccagcagttctgggccagctgagggactgggggtggtgaacaggatgccctggggcacaggtagctgctctgctggttccaaagtgggcctgggcacagccgagggcacctccacccccaggtctcccgccagtagactcagtagagcatccccagcaaggtctgaggtgggagcgagggctgcgctgcgaagcacagctgccagttgtgggttggtggctcgggccccagcgcccaggggtgtcccatcagcatggcaaagtagtggacagaggccttctgtgccccgagccaccagagcccttgccaggggtgtgtccaccaggaagccctcctgagccagcgtggtggggcccactagcaggcgtggccagggcaggcggccgaagcgtgcatgcagcaggtgcagggtgggcagagccgcgggcagccccaggccgggggccagggtctgtgctgggcctgatgtcagggccgtggaattgcctgaggagctatcgtggaagaggccccaaaacatggcacctagccccgtggcatgaggatgcaccactgccaggcacaatgcagctccaactccagcatccacgacgttgcccccggcaacaagcagctctcggcctgcagggctgatgatggcaccgtggtggtatacgccagggccgtgggagtgtccgccgggtggaggggccacagagcccaagcttcctgtcgacctgccctgattctggagctgcctcacagccagggagcagccaacagccagcagcagcagggctgccactacacgggcccaggttccgggcagcccgccagccttgttcctggaagagtcctggtgcctccgggggtttagaaccagcgcctctgatgtctcctcctcctccacttcctcctccgactccaagcttggctcccagggcagcagcttctgatagaccacgggctcttctgcccgctccatggccccccagtgctcgccccagccctcctgcctgccagcctttccggctgtgtctc

SEQ ID NO: 14020 - RNA, 1877 nt, Homo sapiens
  source 1..1877: mol_type = other RNA
gctgggattacaggcatgagccaccgcacccagctatttttttattattattattattattttaaagacaggttctcactctgttgtccaggctggagtgcagtggtgtgatcctagctctctgcagccttgaactcctgagctcaagcgagcttcctgcctcagcctcccaagcagctgggacaacaggcatgtgccaccgcccctggcaaatttttaaatttttagtacagatgagatcttgctttgttgtctaggctagtttcaaactcctggcctcgaggtatcttcctgccttgaccacccaaagtgctgagattacaggtgtgaggcaccacaccctgcgggtgcacactccattgctgctgtgtctgctctgctcctgcccccatgcttcagataactctgccttctgccagacccacccccatcctgttagaacccctggaaggggcagcaggcatgggggacactggagacatgggcgtgctctgtgtgggctgccacctggagcagggtcccttggccacaagtgctgggatgctctgttggttcttgctgaccctgatgctggtgctgggcctgggtagggggccttgctgccagatgcctgagtagggtgtgagtcatggccctggccacatcaggggtccctgaagccacaagccccaacacatcagcctctgtgtcatccaggctgccacggaggatgagggggcaggcccaggcactagtggtagacttggccaccaggttgctgagcagaaccccagtgcttggggacaggtgtgcagagccaaaggagcagttgagcgaggaggtgagaaggagcacagagccgctgctgtccacggcggccagggcactgctctcggggctcacagcagtctgcaggaacggtgggcaggggtcagggatgggcgccccggagcgcagggctgcctccaacagtgccagcagttctgggccagctgagggactgggggtggtgaacaggatgccctggggcacaggtagctgctctgctggttccaaagtgggcctgggcacagccgagggcacctccacccccaggtctcccgccagtagactcagtagagcatccccagcaaggtctgaggtgggagcgagggctgcgctgcgaagcacagctgccagttgtgggttggtggctcgggccccagcgcccaggggtgtcccatcagcatggcaaagtagtggacagaggccttctgtgccccgagccaccagagcccttgccaggggtgtgtccaccaggaagccctcctgagccagcgtggtggggcccactagcaggcgtggccagggcaggcggccgaagcgtgcatgcagcaggtgcagggtgggcagagccgcgggcagccccaggccgggggccagggtctgtgctgggcctgatgtcagggccgtggaattgcctgaggagctatcgtggaagaggccccaaaacatggcacctgcagggctgatgatggcaccgtggtggtatacgccagggccgtgggagtgtccgccgggtggaggggccacagagcccaagcttcctgtcgacctgccctgattctggagctgcctcacagccagggagcagccaacagccagcagcagcagggctgccactacacgggcccaggttccgggcagcccgccagccttgttcctggaagagtcctggtgcctccgggggtttagaaccagcgcctctgatgtctcctcctcctccacttcctcctccgactccaagcttggctcccagggcagcagcttctgatagaccacgggctcttctgcccgctccatggccccccagtgctcgccccagccctcctgcctgccagcctttccggctgtgtctc

SEQ ID NO: 14021 - RNA, 1287 nt, Homo sapiens
  source 1..1287: mol_type = other RNA
gctgggattacaggcatgagccaccgcacccagctatttttttattattattattattattttaaagacaggttctcactctgttgtccaggctggagtgcagtggtgtgatcctagctctctgcagccttgaactcctgagctcaagcgagcttcctgcctcagcctcccaagcagctgggacaacaggcatgtgccaccgcccctggcaaatttttaaatttttagtacagatgagatcttgctttgttgtctaggctagtttcaaactcctggcctcgaggtatcttcctgccttgaccacccaaagtgctgagattacaggtgtgaggcaccacaccctgcgggtgcacactccattgctgctgtgtctgctctgctcctgcccccatgcttcagataactctgccttctgccagacccacccccatcctgttagaacccctggaaggggcagcaggcatgggggacactggagacatgggcgtgctctgtgtgggctgccacctggagcagggtcccttggccacaagtgctgggatgctctgttggttcttgctgaccctgatgctggtgctgggcctgggtagggggccttgctgccagatgcctgagtagggtgtgagtcatggccctggccacatcaggggtccctgaagccacaagccccaacacatcagcctctgtgtcatccaggctgccacggaggatgagggggcaggcccaggcactagtggtagacttggccaccaggttgctgagcagaaccccagtgcttggggacaggtgtgcagagccaaaggagcagttgagcgaggaggtgagaaggagcacagagccgctgctgtccacggcggccagggcactgctctcggggctcacagcagtctgcagggctgatgatggcaccgtggtggtatacgccagggccgtgggagtgtccgccgggtggaggggccacagagcccaagcttcctgtcgacctgccctgattctggagctgcctcacagccagggagcagccaacagccagcagcagcagggctgccactacacgggcccaggttccgggcagcccgccagccttgttcctggaagagtcctggtgcctccgggggtttagaaccagcgcctctgatgtctcctcctcctccacttcctcctccgactccaagcttggctcccagggcagcagcttctgatagaccacgggctcttctgcccgctccatggccccccagtgctcgccccagccctcctgcctgccagcctttccggctgtgtctc

SEQ ID NO: 14022 - RNA, 3544 nt, Homo sapiens
  source 1..3544: mol_type = other RNA
gctgggattacaggcatgagccaccgcacccagctggaactctattttcaaatatcattttctagaactcgtattctactggttacaatttggaaaatgctagactaagtgatccccaaaggcctccaagcattaatattctaaaattttactctctgattcttttcttccccctttaatcctaataaggagctccacatgagattctgcatatccaaactctttgcaaacttaaaaataccaaaaaactgttagctattataacatgggggcaggaccagggagatgaagcgtatcctgtcaacaccctgagaacatgggtaacagtctccactagaaaatctctgacctgcaattatgtctttttgtaatgtgcttaattacatacttagaaaataaattctagaattccagcacaatttttgtttaaggaaataagaaaatcctttgttttgcataaacggtgttacaactaattaagggagaaattagctgccaggttacatgaaaagataagacctgattccatgacatcttctttgcattcatgagaagcgagctgatggtctgctgcctgtgtggtgtttagctcagcctccactgactgggactcattagccaagggttacaaaaaatgtaaccaatgctttttccagatattccaccgcaaaccaagtaagacggtgtctgtcccttgccttgaaggcctgggtctgagccactcacgatgctccctccagctcagcctgcggcatgggattttcattagatggcgttccttgtattcaagcaagtcctgctggggtataaataccgctccttatgaatgggattagtcctcttatagaagagacctcagagaggttcctgactccttccactatgtgaagttacacagagaagacacatctttgctccagcagattctgaccgtcataatgatcattccccaagtcatcaagcacaatgcaacatgatagagctggttataccttgatgagaactttccttaaaacagactccaatatttccatacaatggcttacaacaaaactctctgaaggaagtatgccaggattggtttttgatatttacagttgctgaagtaatcgcttcttccttggcaaaggaagaaagttaactcatcgtggtcttcaaggcaccttctagggctaacattttatgactctgttgaacagaaaacttttcagaaggcatctgccgaataacatgaataaaaatgcttcaaaggctagttacaaattttaagtactccatactctatttttgcctcttttccttctgtttcttaccctgtattcatttttcattaatattgctaaacaaagaggagagaaagagaagttttattaagtcaaatttgatgggatagaaagttgaagttctgagattatgcacagaattttcccacgtttagattctctgaaatatgtctttcttcagtggctttgaacaggaagagttagctgtgatttgaaccttagcaagcttaaagattggttgtaaaagcacctctaaaggagaatgctggcagaaaatgcaatgaacttctgctagagacctcaacacagctgagaatctggaaatttgtgctatttgtgataagaatttaagcaaccaaaagtcttttgttttttgaaaatgaaacaaaacaaaaagcagcgacttgcaagtatacaggaagcttatctccttcagttcaggagtatttgtttgccaactaagggttacttttcacaaatgtaaagttaagtcaacaactttcttggcatttatgacactatatataaaagagcctgtgaaatatgaaatgaacttttcaggttttgaaattgatacaccaagattaggaaaataaaccgtttgatgagtgttttgctggctcatttaaactacattcccagtcataactcttgatttcccaagcaaggaaacagaaagagaaagagaacacagtatgttctgaacagaactgagtgctccttgcatgacttaggagttagatccacgtgaaacatttatgcttaccattacttaccactcccattgttactattattaatgttgtacattagaattaagtagtttccagagtgctttcatatatttttttctcatttttacatgacttcccaatactgtgatgtagattaaacaggaagtattcagatatattaagtaatttagcatccatcaccattatcatcaccatcatcatcatttaatgagcacttactatttgctaggccctgcactcaatgtcttatatgaatcatctcagttaatcttcacaacaattctatgcaattggcattattattgtctgtgttttatagaagagaaaacatggttgattgggaactggaatctggagcttatgagaccaatttcagtgttctctccatattgttttaataagagtttaaaaagaacaaagagaatcctaaagtttccagttcatttcatatcagtttcttttagacataaataagacaagaaagagaccatgaaaagaaggttaaattttcagcctcttcccaaaataaatacttacaaaaatgcaataggcaaaaatatttgccatatcttttggaattttgtaaattgcaataaacttgcaattccactgtatttgcagctaaatgcaaaattctacatttaatcctgctactgaccaaaccatgtctttttgttaaaaaaaacaaaaaaaaatgtctctgttaaaaagcctgacagtgtggtgtagcctaccatgactgataaagctcttgagcttccaaaccagcctggttgcagcttggttggtctttaactaggtcagattcaatttccactcagtaagtctttaatcagtgtctactacatgattggtgtcaggagatgtggaagtagacagaacactggttgtttctgctcttctgaagcttacaatcagaccaagacagatataagagatgaattatagtgtagtttcacaacagaagatttatccttgtcttgggacttacaggcaccttccctgaaaaaaaaaatggcatttagatgatacctgaaggaatgccattagtctgatggagaaatggcatgaggactaggagacattcacaaacttaagcaaaatttacatcccccatgagatgaaggagttttccataacctactacaaggtagaggttttgaaagagaagaggttaatatataaaaagtcaatctttaaaacattttccttggtcaagaattctcactctgaagaacctagtttataactgcctattctggaaggagggtgaaagcaacacactactgatggtatcttagctaattgcaataatggtttcatcagcatcagggaaaaaaagtagggtatgtatttaaaagcgcataagacaagaaagtacagattgaaaaaactgattggagaaggaataaaaatagagaaaagggaggaatactctaaattaaatagaattatagtaagaaaaactaaaaattttactatgatgagctctcaattacttgcacg

SEQ ID NO: 14023 - RNA, 2698 nt, Homo sapiens
  source 1..2698: mol_type = other RNA
gctgggattacaggcatgagccaccgcacccagtcaaactcttttatctttagtaagggtagaggaccagtcaaagcctttgccacattcttcacatttgtagaaattctcttccgcatgaattctcctatgtgtagtaaagtatgagtactggttataaggtttgccacattttttacatttgtagtgttattctccaatatgaattatcttatgtatagtaagggttgaagattggttaaaagctttgccacattcttcacatttgtagggtgtctctccagtatgaattttcttatgtttagtaaggtttgaggaccagttataagctttgccacattcttcacatttgtagggtttctctccagtatgaactctcttatgtctagtaagagttgaggactggttaaaagcttttccacattcttcacatttgtagggtttctctccagtatgagttatcttatgattagtaaggtttgaggatttttaaaaagctttgccacattcttcacatttgtagggtttctctccagtatgaattatcttatgtctagtaatttgtgaggaacagttaaaagctttgccactttcttcatgtttgtagggtctctctccagtatgaatcatcttatgtgtagtaaggtatgagaattggtagaaatctttgccacattctaaacatttgtagggtttctctccattatgaattctcttatgtttagtaagggttgagaatacattaaaggctttgccacattcttcacacttgtagggtctctctccagtatgaattatcttatgtttagtaagggttgagaatacactaaaggctttgccacattcttcacatttgtagggtttctcaccagtatgaattctcttatgtgtagtaaggcgtgagtaccagttaaaagctttgccacattcctcacatttgtagcgtttctctacagtatgaatcatcttatgtgtagtaagataagataatcggtagaaagctttgccacattcttcacatttgtagggtttctctccagtgtgaattctcttatgtgtagtaaggtaaatgaatcggtagaaagctttgccacattcttcacatttgtagggtttctctccagtatgaatcaacttatgtgcagtaaggtaggagtaacagttaaaagctttgccacattcttcacatttgtagggtttctctccagtatgaattatcttatgtgtagtaaggtatgagaatctgaagaaagctttgccacattctccacatttgtagggtttctctccagaatgaattttcatgagtagtaaggtttgaggactgtttaaaagctttgccacattcctcacatttgtagggtttctcttcagtatgaattatcttatgtctagtaagggttgcgaatacattaaaggctttgccacattattcacatttgtagggtttctctccagtatgaattatcttatgtctggtaaggtgtgagtaccaattaaaagctttgccacattcctcacatttgtagggtttctctccagtatgaattatcttatgtttagtaaggtatgagaattggcagaaagctttgccacatccttcacatttgtagggtttctctccagcatgaattgtcttatgtttagtaaggtgtgaggactgtttaaaatctttgccacatttttcacatttgtagtgtttctctccagcatgaattaccttatgtctagtaagagttgtggagtggttaaaaccttttccacattcttcatgtttgtaggatttgtctccagtatgaattctcttgtgtctagtaagggttgagaaccatttaaaggctttgccacattcttcacattggtaagaattctctctaatatgaattattttatgttgacctaggtgtaaaagcatgcaaaatgatttgccacattttttacatttgaaaggtttctttccagtatgtcttgtcttatgtgtatttgaatttaaaaatttatgaaagactttcacatatttatcacattgaaatattttgctctgggtagttgtcaaatactcttttagttcattataaccttctttttgcacattacactcattcacacttttacagccttttcttaactgtaaatctttatgtccataatttccatattctctcagtatcactttttggaaagaatcttttatgcccggctgtggccaaaggtcctgggcaaaatgagaatatgtaactgggggtgtggctaccatactgtgtctcttcatattccagggatcttttccttgctccagacaggtgatcagatctggcttagagacatcaatacccaagaacaccaggtttctgaagttctctaacatcactttcctatacaaatcttgctgagcagtgtccaggcattgccactcctcctgagagaattctatgaccacatccctaaatgtcaacggccccttttcaaaataagagtactccagaagattcctctcagccccagggtatccacttgcccccttgacaggatacactccatacctcaggtcgtccatttctaggcttccagggtgtcccggcgtcttagctgtggattcccaatacctgcaggtcacaggaccagaggctgggcctctaggagcagaggacacagagcagtgaagacgagacccggagttccagcggcagccaaagac

SEQ ID NO: 14024 - RNA, 2804 nt, Homo sapiens
  source 1..2804: mol_type = other RNA
gctgggattacaggcatgagccaccgcacccagtcaaactcttttatctttagtaagggtagaggaccattgaccaggtgatctgcctgcctcagcctcccaaagtgctgggattacaggcatgagccaccgcacccagtcaaactcttttatctttagtaagggtagaggaccagtcaaagcctttgccacattcttcacatttgtagaaattctcttccgcatgaattctcctatgtgtagtaaagtatgagtactggttataaggtttgccacattttttacatttgtagtgttattctccaatatgaattatcttatgtatagtaagggttgaagattggttaaaagctttgccacattcttcacatttgtagggtgtctctccagtatgaattttcttatgtttagtaaggtttgaggaccagttataagctttgccacattcttcacatttgtagggtttctctccagtatgaactctcttatgtctagtaagagttgaggactggttaaaagcttttccacattcttcacatttgtagggtttctctccagtatgagttatcttatgattagtaaggtttgaggatttttaaaaagctttgccacattcttcacatttgtagggtttctctccagtatgaattatcttatgtctagtaatttgtgaggaacagttaaaagctttgccactttcttcatgtttgtagggtctctctccagtatgaatcatcttatgtgtagtaaggtatgagaattggtagaaatctttgccacattctaaacatttgtagggtttctctccattatgaattctcttatgtttagtaagggttgagaatacattaaaggctttgccacattcttcacacttgtagggtctctctccagtatgaattatcttatgtttagtaagggttgagaatacactaaaggctttgccacattcttcacatttgtagggtttctcaccagtatgaattctcttatgtgtagtaaggcgtgagtaccagttaaaagctttgccacattcctcacatttgtagcgtttctctacagtatgaatcatcttatgtgtagtaagataagataatcggtagaaagctttgccacattcttcacatttgtagggtttctctccagtgtgaattctcttatgtgtagtaaggtaaatgaatcggtagaaagctttgccacattcttcacatttgtagggtttctctccagtatgaatcaacttatgtgcagtaaggtaggagtaacagttaaaagctttgccacattcttcacatttgtagggtttctctccagtatgaattatcttatgtgtagtaaggtatgagaatctgaagaaagctttgccacattctccacatttgtagggtttctctccagaatgaattttcatgagtagtaaggtttgaggactgtttaaaagctttgccacattcctcacatttgtagggtttctcttcagtatgaattatcttatgtctagtaagggttgcgaatacattaaaggctttgccacattattcacatttgtagggtttctctccagtatgaattatcttatgtctggtaaggtgtgagtaccaattaaaagctttgccacattcctcacatttgtagggtttctctccagtatgaattatcttatgtttagtaaggtatgagaattggcagaaagctttgccacatccttcacatttgtagggtttctctccagcatgaattgtcttatgtttagtaaggtgtgaggactgtttaaaatctttgccacatttttcacatttgtagtgtttctctccagcatgaattaccttatgtctagtaagagttgtggagtggttaaaaccttttccacattcttcatgtttgtaggatttgtctccagtatgaattctcttgtgtctagtaagggttgagaaccatttaaaggctttgccacattcttcacattggtaagaattctctctaatatgaattattttatgttgacctaggtgtaaaagcatgcaaaatgatttgccacattttttacatttgaaaggtttctttccagtatgtcttgtcttatgtgtatttgaatttaaaaatttatgaaagactttcacatatttatcacattgaaatattttgctctgggtagttgtcaaatactcttttagttcattataaccttctttttgcacattacactcattcacacttttacagccttttcttaactgtaaatctttatgtccataatttccatattctctcagtatcactttttggaaagaatcttttatgcccggctgtggccaaaggtcctgggcaaaatgagaatatgtaactgggggtgtggctaccatactgtgtctcttcatattccagggatcttttccttgctccagacaggtgatcagatctggcttagagacatcaatacccaagaacaccaggtttctgaagttctctaacatcactttcctatacaaatcttgctgagcagtgtccaggcattgccactcctcctgagagaattctatgaccacatccctaaatgtcaacggccccttttcaaaataagagtactccagaagattcctctcagccccagggtatccacttgcccccttgacaggatacactccatacctcaggtcgtccatttctaggcttccagggtgtcccggcgtcttagctgtggattcccaatacctgcaggtcacaggaccagaggctgggcctctaggagcagaggacacagagcagtgaagacgagacccggagttccagcggcagccaaagac

SEQ ID NO: 14025 - RNA, 16969 nt, Homo sapiens
  source 1..16969: mol_type = other RNA
gctgggattacaggcatgagccaccgcacccagtcaatttctaagtatttgatggttttcaccacattaatctaactcaaaactgcagctgccatagcaccactaaaatcatttggtttttgaaaagttatgcttttgccaaggattattataaagaaaaattcagcctgtgtgctggatatcttgcagggaagaaacaacaggatatgtttgtaagtgaacactacaccatgataaggcctatgtttctcttattcctatttcataaaatgatctacaacaaagacattttcacagaggcaaactggaaaggaatccttcacacaacactcttctattatcttgaacgtctgaatagcttttcctttggagaactcaaatgcttccgcaaacattatcttattcttacaacaatttagtgatcatgcctataatcccagcactttgggtggctgaggcaggaggactgcttgagctcaggagttagagatcagccttggcaacatgtgagaccccatctctgcaataaaagaaaataattagctgggtgtggtggcatgtacctctagtcccagctacttgggaggctgaagcaggaggatagtttgggcccaggagttggaggctgtagtgagctatgatcacactactgtagttcagcctgggcaacagagtgagaccctgactcagaacaaaagaactccaacaatttagtgaggtaggtgaggacaggtattaccactcttatttacaaggggaaactaggcacacagagattaaacgaattgcctaaggacacggagcaaatcagtgggagacctattactaaattccaagtctctggctcatattctagagccctttctactctcaaaggcaataaattctcaataggctttttccatttgtgatctttcaaaagttcctccattaaagaacaccttaagccttctctcttatagcccacgcttgactaggaactgggatgagttttaaactatttttacacaatattttgcacatatcaagaaggcagatgtgagacataagctgtataataaagtcagaataaatacataaattaagagaaatgaacaggttaagtattaattcattcaatataattttttacatattttagaagccatgtatcagaataaaagtcataacattttaaagtttaaatcagagtccaatttatcaaaaccataagctatattaattttctttaagaatatgaggatctctgttggttggcagaaggttagaatattactttcaagaataattcttatttatttatttattttaaagattggggtcttgctgtattgcccaggcttgctttaaactcctgggctcaactatcctcctgcctcatcctcctgagaagttcggactacaggtgcaaaccaccacatctggctaatatcaacaataatattatcactgtgccataatacatcatattcctgatatatactctgttcacattagcattctatagccagcaaaaaattccatggctagagataatacttgcaacattaatactttcaatcttaattctcacttaactgagttagaatttctcttcatatatgttaaagttacattgtaataatcatcattctatctatttttgttttatccttcccctcttttatttttaacagtgtgtgtgtttgtgtgtgagtgtgtgtgatggggaaaaaagaacaattgtgtgattcacaaatggcataaaacactgattgtattacaaataagaatggtggcactctagtaagtaagataatggaatgtcaaaggaaacaaactttagaatacaaacatggaaaacatgctaaaatattaatcaagctatagcttgtggcatgtgattcttctttcccaagtattttgagagtgtcatttacccccagtagaattctatatcaactgcctctaagtccttttcctattccttcttttttttttttttgagacggagtctcactctgccacccaggctggagtgcaatggtgggatctcggctcactgcaacctccgcctcctgggttccagactaccttgtctggaaaggccctgcttggtgttttctatttaaaggggaaaaccaaacatgttatgttgatagcaatgcctggctctattaaagataaatccttcatttaatttccttattgtaattcagactagcaggattctcctgcctcagcctcaggcgcctgccaccacgcctagctaattttgtatttttagtagagacagggtttcaccatattggccacgctggtctcaaactcctgaccttgtgatccacctgccttggcctcccaaagtgctgggattgcaggcatgagccactgctcccggcctattctttcttttttaaagagggaatggggttggaccctgggctaagaaatgagaaagctcctggaaaaccttaattgcaattaattactatagaagatcaagtctgttgctagcaaaaccaaagcttccttttgttaaactccctgggatcaaactgtatccatgaactgggtcggactgtctatgccaaaattctttcttcattacaaactaaccagtgtttttaccaaatcccacaccaaaaccattttctttacaggaaagactacattgtctggaaaggccctgcttggtgttttctatttaaaggggaaaaccaaagacactatgttgatagcaatgcctggccctatttaaggataaagacttcatttaatttctttactgtaattcagaagcaacttccaagacttctctaagttactgagaataggtgtgcctttgggtctgggacaacattatcatataaatttagattacagagacgctcgtcttaggtctcttctgtaggttcaaatagcaatagctgctcttttactctgcaaatattaaacaattgtaaggtttctgtccaaggatcccagcaaggaagccttatcctaaatcccccctcactatatattctcacaatcctactagtctatttctttacaaagacctccagtttctacagattctgacaataaagagtcacgtatgcaacatttttgcagtctttccttctttggttctaaaaagactattaaaggactaacttaagagatttttgtttgttttcccaaccaaaaatgaaataaagatgaaataaagccatgaaataaagatgaaagttttgtcttttatttttaaaattattattattttttgagacggagtttcactcttgtcgcccaggctggagtgcagtggcatgatctcggctcactgcaacctccgcctaccgggttcaaacgattctctcgcctcagcctcccgagtagctgggattacaggcgcccaccaccatgcctggctaatttttgtatttttagtagagacgggttttgccatgttgtccaggctggtctcgaactcctgacctcaggtaatcagcctgcctcggcctcccgaagtgctgggattacaggtgtgagccaccgtgcccggccaagatgaaagttttaggcactaaatatcagagtaatctccctctctagtctctggtgttgcctcttcaacatcaaacataaaattatagatagcataccgccaatttttggaaagaataaaatttaaaaagcaaggctctaatgaccaacacttccatctgttttctacgcataacgctgttcatggcaattcttttttgggatgatctattactgcacaacgatttttttttttttttgagacagagtctcactctgttgcccaggctggagtgcagtggcacgatcttggctcactgcatcctccgccaccacacccggctaatttttgtatttttagaagagacagggttttgccatgttggccaggctggtcttgaactcctgacctcaggtgatctgctcacctcagctgcccaaagtgttgggattacaggtgtgagccactgcacctggccacaaagctttctttctaaagaggtgaactaaacatgaacaagccatcaagtacttcactgcggtcaagctgtactgatgtcaggtagcaggatttgtggagccaaccagttaaaacagcaaaataagctctatatgccaggtttctatgaactttcagaaggaaaaagaaaacacaggaccagaggcacctttttttgtttgtatgtttgttttgagatggagtcttgctctgttgccaggctggagtgcagcggtgcaatcttggctcactgcaacctccgcctcccaggttcaagtgattctcctgcctcagcctcccaagtagctgggactacaggcgtgtgccaccacacccagctaatttttgtatttttagtagagatggggtttcagcatgttggccaggatggtctccatctcttgacctcgtgatccgcccacctcggcctcccaaagtgcagggattacaggcgtgagccaccatgcccagcccagaggcaacttttaaaatgttggttttcaggaactacatgtctgctaaccttggacatgttgaaatgtaatgaatacaactattaaggttataagcgcaataaatatccttaaaaggggacatacaatcacagcaaaaatattttgctttttttttttttgagacggagtcttgctctgtcgcccaggctggagtgcagtggtgtgatcttggctcactgcaacctccgcctcctgggttcaagccattctcctgcctcggccttcccagtagctgggattacaggcacgtaccgccaagcccagctaatttttgtaattttagtagagacagggtttcaccatattgggcaggctggtctccaactcctgacctcgtgatccgcccgcctcagccgcccacccaaagtgctgggattacaggtgtgagctaccacgcccagccacattaatttgcttttaattagtagtaacaaattcttataatcagagtacaaatctgtactatctgtatacaattagtacttgatgtgtgcggggctgaagtatctcagaatagtatatcatagggcaaactaatgtaactggcaaaaatgcaaaaagaaatgaaatggctaatctctacaagaaatcacatgctgatctattttaaactgtaaaactttacatcatataaaaataaaattttcccatttataattacctgacactttcccatttccttgcctctcagtggaatacactacagtaaaatgtcatacattgagctccaataatttagaattgaaaacccagaggatggaatacagtttatcttttaaccacttacagaaaagaaatttcttaacaagcaaattcatgatgtaaaaatacaatgcaagtattttacctgcttaagggaatatacttttttcatgtacttttatttatttttatttttattttctgagatggagtttcactcttgttgcccaggctggagtgcaatggcgcgatcttggctcactgcaacctccgcctcccgagttcaagtgattctcctgcctcagcctcccgagtagctgggattacaggcatgtgccaccatgcccagctaatttttgtatgtttagtagagacggggtttcgccatgttggccaggctggtcacgaacccctgacctcaggtggtctgcctgcctcggcctcccaaattgctgggattacaggcgttagccactgcgcccagcccatgtacttttattttaaaagttaacataccaatatccataatcttgatcttggccagatgcagtggctcatggctgtaatcccagcactttgggaggctgatgtgggagaagcacttgagcttaggagttcaagaccagcctgggcagtatagtgacccccatctctaaagaaaaaaaccattagctgggcatggtggcgcatgtgagtagtcccagctacttcagaggctgaggtgggaggatagcctgagcccaggagtttgaagttatagtgaactatgatagtgccacaaaacaaaacaaataatcttgacctattcactaggaaactggactgtctatatataattgaacttaatattctataatcatgctttttgctgccttccaatttattcacattcataaattattactatttaaatttttaattagctgaagtactctattaatcagtctttatacctggctctccctagccacttaaactctgatttcttcattgatactcagggattcaatcaactttagaagtatgctagggaaaagatcagggtagcaaatcttccatataacaaattatgggggaaaagtttcatttcaaagtcaattcaatgaattttgaatcatttgctatttgttttccaggcctacaaaaatggtatcttaatcctaatgctgaaaaatgtgaccatttaagcagtttcaatgtgcttaaatttaaaaaaaaaaggcatgtaacaattatttatttgacaggtttccccaaaactgtagtcaggtaaaataaatccaatctgttatgttagtttgctactaaaggggaaaaaaaggatcaaacttacaggaaagccccacctcccctccacatgtagaaatctgtctaaagactgtctttaatgcccactatataaacaacattaaatattctaagttacaaaatagtgttaatggtttattggtaaaaatccaaactctagagtttatggaattcgtagtttggttggtatattaacactccatcttaatctttgctgctattacaaagaatgaggaaagctagaaatatctataaaaataaaataccttaaaaccgacaagcaaaatataaaagttgcatacaaattgccaataaatataaacatcacaatagaaaaattaatcttaacaaaaataaactcataattgctattaagacattataaaaacaaaaaagtttaatgtgcatgtatatttgcaaacagacacagtacactccaaacaatataattttactatcattattatataatgcagcatacaaggttactgaggtgtggtattttttgttgttgttgttgtttgcttttagtcttcttttctggaagaatgctcaccaaattcacaggaaagaagtgcctaggtgatcatttactgctatttactgcttcctggtatggagcaaaattgccctctggtaggtaactacatttctaattagtatgaaaggttctactattttcctttcttttgcttatttccccttaagcacaatttgcagaccctacttctatttaactgatcatacccttttaaatgccttgtcatcatttttcatagttcctgcatcctagaaaaaataaaaaatcatttaaaatattccttggtgtctagaaaagaaaatttctctaacaatagagattatcattttgctttctcacttaagctgatctgaatgatgatttggtactgcctttatgagcagtcctccttaataatgactaattagggccgggtgtggtggtgcatgcctgtaatcccagctacttgggaggctgaggcacgagaatcacttgaacccgggaggcggagtttgcagtaagctgagattgagccactgcactccagcctaggtgacagagcaagactttgtctcaaaaaaaaaaaaaaaaaaaaagattaattagaaaatgttgcctatgattccaggcaagttacatttccctttggacattggtactatacccataatcttgttaaaaagttaagtaggtttgctgttttatgtgcattatggatttcctccaacacagttgggaattaaaagaggtaattctactaaatattttgttttcaaatttacaaaataaatttggtgagcatttacctagatactttactgcataaaagctttccttggttcccttggacgagattcaagacaacaactaacattatttttatgaaactgtcacactcttggagttctaaaataatttatctttaaaattcttagcttcgtgctacttgaaaaataaaaatctacagcaccatcttctgaaaaggcactttctaagaaccgccttgctttaaaaaatgattaaaaaatttaactcaagagtctacgccctgacaaacgtctttgctttactgagaccctaacatagatacattagattctggttaccttagaaattagtctaaaaaaggaagggaccccgatggctggataggtgatttgacaggattctaattttgtcacaccatttacctgatacttcaacagggtttctcactggtaaatctcaaccctctatattgaatttaccatccttctatctttaattcaaattaaaatctttaacttccatattttaagaacaaaagattcttgagatttaatcaatgatgtaaacatctggagtactagttttgatgggtaaagtaatataaatttcaatgagtagtaggtaatattagcacaagccttgaccattataccttagtttaaaaaattatgttgactgacatggaaaattataaacttaaatgtaccattttaaaagtaggaaaaaagtcaaaataatttttccctttgtgtgtgtgtgtgagattatatatatacacactcatacatatacacacacacacactccccctccctgcttcctgggactcagcttggctttcactaatcacagtgtcatttctaacactgcaacggatcaagaatgttcttagtataagcaggacttttttaaaaagattttttggagaaaattctcactttctgatttctgtgctgactgacttacctactcttggctgattttttgactcctatagaatcacaaaagtgcttttctatgatcaaatatgaggactgaaataggaaaacaagagttctaaattagggttatactgctacacaggaaggcgttacttgatgtcaaacctcccaacaattcttactgaagctttaagacatttatgaattctcaaaaagaatgaaaataatgaatacttcatatggataaagccaaaataaagacgccacactaatgatatttttgcagcttgactaactaataaaaggtaatttaagtagcaagttactgttaagggcaacctgcctgttcaacagaagaacatctaagaggataagctaagcaaacatttaactcaggtttaatgatactgaatgaaaattttgcagagttgtcagttaaacttcttggtaaaaatattaaaatcaagtttgaaataggaagactgcaacatattctagctgtatcgaagtcgtttgcttcttgaatttcataaaaatcactgcccttggcaaattcatgtagggctctaaacagatccatcaagttccttgagtcacaaacggtctctaattcctggtctgcaatccatctaaatacttcggatccatcactggcatgcttagcgctcaccctttccttgaacacagagatccgctgccagtcattcctgctgaagggcaagtcaggttttatttccctagacatgccttcagtctttcatgactctgtcagaaggcctatcctcctaaaatccattagagaatacacaagcaaacactaggcagtggtgggctgtggagaagctagcttggaaactggtctagatctttagaaggctgagaatccctgtgctggaaagcagagatgcctctatcaagtgccttccaaaacactcagtaattcctactagaatccctgctagactctcttctaggaatagaaatatattaataggttataaacagggatttcccttagaatgatagtttttccaagaaacttgttagaagatcactattaagaaaaagaaagggaatctaatatttctgttgaaatgtgccaaaaaaccagtactgaagaggctgaggtaccctttttcaaactgtaaaagtcaaaatctacatttctaaaacaaagaatatcctgatattaaattgaaactaaaatggcagcaccctttgttactttgatattccgtgtccttactcttaggaaaaaaaagggtctaacactagccttgaatcctgcttatctccttactgtttagtgcagtaactgtcagaatctacttaaataaatatagcagctacaatattgtaagtgtatggtcctccatgccagtaacctgatactgtgatataatacatgtatcagcactttatgtagacacattaaccatcaagaatatacattaaactcccaactcttcttcatatgaaaatcaattatctagttgccagactgatattttacagtcagtctcgtaagatacatcacagaaaaaagaagaccaaaatctagcattcatgatatagttagtgagcaagggcaggagcagaagggtcactgtgaatttcatgtttaacttaaaaaaaaaaacttttttaaaataaaaaagattagaaattctacaccagaaatgcaacaataaataggacaaatttcaagaagcatttgtcacttagccttttatcttaaaattctaagcacaagttttcttgtaattaagaaccaatggtaattaatataccaatttgttagcaaaatagaaatatagtatacatactctttcaagttaatcaactttaaactagcaatgctgactagtgtaagagcactctaaaaaagaaatcactcaaaaggtaaagctttataatttagaaaaaatatttttcctcttaaaaaagtccttccaaatagatttaaattaagggctccactctagcatatatgagtgactgaaaattaggtgagagagtacatagagaaagggtatctacagtcattccctaaagtttcccacatgaatctgtgcagctcccatgataaaggaagatgttttactcacactgatcaagcatagacgaattaaatttttatcatcttgggtatactattttcttctcttgcccatgatcctgactatattcagtaaaatttcagtgtaaaaaaatccatctttataggaaatttttctggaggagatgggagaaggctgggagaaaaaatgtatatacgatacaaatattaccttttgtaaagttctttgcaacagtgttgtaaattgcatttcagacacttcaaaataataaacatacaaaatacagtactttcttagttttctggcagagggacaaaagatttcatgcctgtcagaggacatgggctcagattttaggctcaaaatacagtgaattggcaataatagtggattacaggtaagagagaaactaaagatctaaatccattaggtttcacgtgcagatggaattctgaaaggctaacaacaatgcccactggaaacaatctgtagtatctatactctgaaccagtgcaaaaaaaaaaaaaatcaaaatgcaattttcatgagttacaaagtgcaaagctcccctgaatccaatgttactgataaactcagttttgatagctttatagtactttttaataccttaaagtgtaatcaataaaagttttgtaaaacaatttcccacgtttcagtgatttaactgatttaaaatgatcaaagtcctaacttcctttgttactatcaccttaattttaaaaggaaagttatactggtgatacattagcaaaagttttaaaatatcatcttgcattttcctgattcattttagtaaatgaaaatgggcatctagccaatatgattcttcaataaacacaatctatttgcaaataatttaaatatgttaagctattcacaattatataaaagttcaactttatttctaatattcaagttggactcatttaggcaatttcacttcattttcattatgatttttttttcttttgagacggagttttggttttgttgcccaggctggagtgcaatggtgcagtcttggctcactgtaacttccgcctcctaggttcaagcaatcctgcctcagcctcccgagtagctgggattagaggtgcccactaccacgcccagctaatttttgtatttttagtagagacggggtttcaccacgttggccaggctggtctcaaactcctgagctccggtgatatacctgtctcagcctcccaaagtgctaggattacaggcatgagccaccgcgtccagccttttatcatgatgaattttaaaagatatgctttaaaactgaaaattacaaaactttccttctgaaattaaggctgtattctttgcccttttaaactatggaggtgcctgttcctcctactatccatggtaaagatgcagacacaactttcctttaaaactgcttattgcactaaaagatagcaaaaacaagttgtcagttcttaaaataaacatgattatatttctataaaagatgctgccaatacaattctataattattaaagcactattctaataaatataaaagaaaaggaagctatacttccaaacacatacatatgtgtttatatacacacacatacatatatatatataaaaaatatatgaaaatcacattaaggtatgagaggcagcaagtaaactatcaaaaaacaaaacaaaaaaatccctcaacaaactcttctctctactcaatttcagaggtctcaaccctacagagctctaatcttttaaaatatttaccctttataaaacctttaaagaatttccatgtataacccatagaaacagaaggcttcagaatacacatcacttaccagagagaaagttacaacttctgacaggttttatatttatagcagctttaacaaactcactaaagaaaaagaatagtaggccgggtgcggtggctcatgcctgtaatcccagcactttgggaggtcgaggcgggtggatcacaaggtcaagagatcgagaccatcctggccaacacggtgaaaccccgtctctactaaaaatacaaaaattagctgggtgtggtggcacatgcctgtaaacccagctactcgggaggctgaggcaggagaattgcttgaacccgagaggcggaagttgcagtgagccgagatctcgccactgcactccagcctggtgacagagcgaggctctgtctcattaaaaaaaaaaaagaaagaaaagaaaaagaaaaaagaaaaagaatagttcaggttgctactgcttatatacaaattgcgcaaatggtaaatgtatgttctgagtgggaggggagagacgcactctcacagaaagttattttatgtatatatatgtgtgtgtctgtgtctgtgtatgtatgtatacatatatatataaaattttgtttcttaagacagcaatatcaagagttgagaactcagaattgtgtatgagataggagtcaggagtagggtatgcaaaataaaagtagaattctagtttgccatattttatattcaaacgaaccagatacatcaacatttgaatgtcactggtaggactgggaaaaaaatgtaggtgatgaaggcaagggaaatagagaaataaaggcggtagtgggggtagaataaaagggaaagaaaattccccaatggaatgaactctaaaatatataacagacacatatatatctattatcaatccagatctagatatatatgcatatgaagtatggatgtatatattttaaaaatacacagacaccttttacaagaatatatgaatgcacattaattttttgcacacataattctgaaaaatcactttgattattcatgaaggtgtgtattttttaaaccatcatttactttttctttacttttttttgcaaagatagttgtgctgccaagcaacttgaggtaaaggcattaaaagggttagactacaagaaatgaaaacaaaacaattgcgatacttcctataggagaccgcacaaaaagcagttggctggtttcatattgcataatgatgctgtgttccttgatgaagtaaacaatcttccttgtattaacataaggatcagaccttggcccccacacagtgttggtttctgtatggctggaggtgtccttactcaattgacttcactggaaacatacgttgtatgtcaattcatctttcagtacttcctctcagagaatatacttggactatttaagcgaagtacattgtgcgtaaggtatcttggtgaatctgtacagccttggcaagagcttgtggatctcgcccattgctttgtcctgaaacgtgacttccttcagcactgtcatgttctttgtccacaagatgatatctggctctaaatgctaccaggtgagcataatacgctggtgcaggtatagaaacagatcgtgtacagcgtacgtaagtgtggcagagctggtaagttagcagctgaagttcatctgcagtaaagcagttatcatcccataaaacatgatagtgtgaaggacgactggtaccctgtattccagcatggctacagaggtaaaaatcgaactcatatgggtgtgtaatgtctgtatcaactgttgttccagctgggatattgccacttcttccaaccctttctgtcctatcagcacaaaataatcgagtgtgatgtctcttctgaactacaatgtaggttattccaggttgatagtctttctccaaactgatgcaggcttctcgaattgctagtagttcataatataatacctgcctaaactgcccctctgaaacaccatcccgataaaagatgatacgagtaggcttgaaccgagttgacttataaaattgaataagaagttcccggaccatggaggccaagtcctggatgatctcctgtcggggtctctgaactcttactgtggcacagtatctgcttgggtgtgcatccatactacctacaacagcagcaatagaaggcttctttccatcaccagcaggtggatgagtgacatcggctcccaaaaagatcactggttgctggaacacagaaggtctttgatgaggtacaagaatattattgatccctccgagtttaacatttatctttaggcacaagtttgacagagtttgaggagatgtttttattacattcttgacttgaacacattgtgtagccatacccaaaagtgtgtctcctacacgtttcacttccgcatacactggtgtcttccccggcaggatgacgataataagctgtaggccagaatatgtgttcttgagatgccggaacatgggctctacgctgtctgccccctgtgcatatttgcagaagcatggctggccctggatgggcatccctgcatccttagaaatcttacgcagctggtctgtgaaacccttcaatatttcttctctgcactgcctctgtgtggcaaaacaagcgatagcccacattttgatttcaactcctgtgtggaattgtttccctcgcatgtcccatactccatggctcggtgttgctactgtccgattccgtcctccatactggagcataggtgctggaagtacgcgtccagttacatgagccatttcatcccgaactttaaattgaaactcctgaacaaatggatctgtttcataatttgcacttcttaccaatctgctaatttcctcttgtctatctggtgcagatcttgctgttgccttgatcatagtggaagtctgattgtctgttagcttcttgatacatcgttgccctgccacaatattacagacttctagtggcaggtaggtgtgtttctgttcctgcccgacttgcagacagggaaggtgcgggtacttcagctgaagagtatacttttctctgaaatactgcgctactgttctctccacagtttggccgttttctaactgtaaaggaaaggtttgatgactggcaggcctccttgttacattacaaacacggtatttccgtctcattgttccacaatgagtcacttcaaccttcaaaccttttatctctttggtgaattttacccgatgagaatcagtcagaggtcttggttgctcatcaatattatgaatatcaagaacttcacacatgaactgaattacaggttgtgctttgtagaaggcagtggcagaaacatcgatattaagcatcattttccacatggcaggccgaacagactgatggaatccaaaccacacttccctgccccctcccagagggtggtcatatccttctggagcggagaaaaatgaacgccccacaggtgtgtatttcatggagggcagatgtcgtagcaccacatcaacggcatggacagggttagtgctgattggcttgtctaattccagtggctcaggcaaggtccgtcctgtcagtacttcatgcagtaggtgccaactcacccgagagacaaatttgattgacaccttgaaaggtcgatcttttccaccttccccaggtaaagtaacgtctaaatctacccctgtagttgccacaggaagtggattggcggtgtaaagacttctttttccatcataaactggtctacggtctccaaatatagttactttaaaatgctgaaccattgagtcaaccacctccctgttcactctcctaggacacttgtctggtttaatatctacctcatagaggtagacatcaatctttgggatttcaacttgaaaacagttagccagcagtttaatgggtttgcccatggtgccatagccaggtcttctgggcaccatgagtaggggctgggccccagcgggtcctgcggagccgatttccattcatggagctggggggagtgcttcgagggagaacggagcccgccactggcggcaaggaggcggcccggggggcgacgcggcgcgacgcgacgggcactctcactcggccccgaggcgggggcggcgacggcttcccctgagcaaccgcactccgaaagctctgggccggaagagtcgcggacggaaaacggcacaggactaggcgagaggaaggggagatgtgaggcgcggacagaggggagtcccgtccggaagttgcatcgcccgcggccgccgacgctcccaccgctcctccacgactgcgggccgccgccgccgacct

SEQ ID NO: 14026 - RNA, 16711 nt, Homo sapiens
  source 1..16711: mol_type = other RNA
gctgggattacaggcatgagccaccgcacccagtcaatttctaagtatttgatggttttcaccacattaatctaactcaaaactgcagctgccatagcaccactaaaatcatttggtttttgaaaagttatgcttttgccaaggattattataaagaaaaattcagcctgtgtgctggatatcttgcagggaagaaacaacaggatatgtttgtaagtgaacactacaccatgataaggcctatgtttctcttattcctatttcataaaatgatctacaacaaagacattttcacagaggcaaactggaaaggaatccttcacacaacactcttctattatcttgaacgtctgaatagcttttcctttggagaactcaaatgcttccgcaaacattatcttattcttacaacaatttagtgatcatgcctataatcccagcactttgggtggctgaggcaggaggactgcttgagctcaggagttagagatcagccttggcaacatgtgagaccccatctctgcaataaaagaaaataattagctgggtgtggtggcatgtacctctagtcccagctacttgggaggctgaagcaggaggatagtttgggcccaggagttggaggctgtagtgagctatgatcacactactgtagttcagcctgggcaacagagtgagaccctgactcagaacaaaagaactccaacaatttagtgaggtaggtgaggacaggtattaccactcttatttacaaggggaaactaggcacacagagattaaacgaattgcctaaggacacggagcaaatcagtgggagacctattactaaattccaagtctctggctcatattctagagccctttctactctcaaaggcaataaattctcaataggctttttccatttgtgatctttcaaaagttcctccattaaagaacaccttaagccttctctcttatagcccacgcttgactaggaactgggatgagttttaaactatttttacacaatattttgcacatatcaagaaggcagatgtgagacataagctgtataataaagtcagaataaatacataaattaagagaaatgaacaggttaagtattaattcattcaatataattttttacatattttagaagccatgtatcagaataaaagtcataacattttaaagtttaaatcagagtccaatttatcaaaaccataagctatattaattttctttaagaatatgaggatctctgttggttggcagaaggttagaatattactttcaagaataattcttatttatttatttattttaaagattggggtcttgctgtattgcccaggcttgctttaaactcctgggctcaactatcctcctgcctcatcctcctgagaagttcggactacaggtgcaaaccaccacatctggctaatatcaacaataatattatcactgtgccataatacatcatattcctgatatatactctgttcacattagcattctatagccagcaaaaaattccatggctagagataatacttgcaacattaatactttcaatcttaattctcacttaactgagttagaatttctcttcatatatgttaaagttacattgtaataatcatcattctatctatttttgttttatccttcccctcttttatttttaacagtgtgtgtgtttgtgtgtgagtgtgtgtgatggggaaaaaagaacaattgtgtgattcacaaatggcataaaacactgattgtattacaaataagaatggtggcactctagtaagtaagataatggaatgtcaaaggaaacaaactttagaatacaaacatggaaaacatgctaaaatattaatcaagctatagcttgtggcatgtgattcttctttcccaagtattttgagagtgtcatttacccccagtagaattctatatcaactgcctctaagtccttttcctattccttcttttttttttttttgagacggagtctcactctgccacccaggctggagtgcaatggtgggatctcggctcactgcaacctccgcctcctgggttccagactaccttgtctggaaaggccctgcttggtgttttctatttaaaggggaaaaccaaacatgttatgttgatagcaatgcctggctctattaaagataaatccttcatttaatttccttattgtaattcagactagcaggattctcctgcctcagcctcaggcgcctgccaccacgcctagctaattttgtatttttagtagagacagggtttcaccatattggccacgctggtctcaaactcctgaccttgtgatccacctgccttggcctcccaaagtgctgggattgcaggcatgagccactgctcccggcctattctttcttttttaaagagggaatggggttggaccctgggctaagaaatgagaaagctcctggaaaaccttaattgcaattaattactatagaagatcaagtctgttgctagcaaaaccaaagcttccttttgttaaactccctgggatcaaactgtatccatgaactgggtcggactgtctatgccaaaattctttcttcattacaaactaaccagtgtttttaccaaatcccacaccaaaaccattttctttacaggaaagactacattgtctggaaaggccctgcttggtgttttctatttaaaggggaaaaccaaagacactatgttgatagcaatgcctggccctatttaaggataaagacttcatttaatttctttactgtaattcagaagcaacttccaagacttctctaagttactgagaataggtgtgcctttgggtctgggacaacattatcatataaatttagattacagagacgctcgtcttaggtctcttctgtaggttcaaatagcaatagctgctcttttactctgcaaatattaaacaattgtaaggtttctgtccaaggatcccagcaaggaagccttatcctaaatcccccctcactatatattctcacaatcctactagtctatttctttacaaagacctccagtttctacagattctgacaataaagagtcacgtatgcaacatttttgcagtctttccttctttggttctaaaaagactattaaaggactaacttaagagatttttgtttgttttcccaaccaaaaatgaaataaagatgaaataaagccatgaaataaagatgaaagttttgtcttttatttttaaaattattattattttttgagacggagtttcactcttgtcgcccaggctggagtgcagtggcatgatctcggctcactgcaacctccgcctaccgggttcaaacgattctctcgcctcagcctcccgagtagctgggattacaggcgcccaccaccatgcctggctaatttttgtatttttagtagagacgggttttgccatgttgtccaggctggtctcgaactcctgacctcaggtaatcagcctgcctcggcctcccgaagtgctgggattacaggtgtgagccaccgtgcccggccaagatgaaagttttaggcactaaatatcagagtaatctccctctctagtctctggtgttgcctcttcaacatcaaacataaaattatagatagcataccgccaatttttggaaagaataaaatttaaaaagcaaggctctaatgaccaacacttccatctgttttctacgcataacgctgttcatggcaattcttttttgggatgatctattactgcacaacgatttttttttttttttgagacagagtctcactctgttgcccaggctggagtgcagtggcacgatcttggctcactgcatcctccgccaccacacccggctaatttttgtatttttagaagagacagggttttgccatgttggccaggctggtcttgaactcctgacctcaggtgatctgctcacctcagctgcccaaagtgttgggattacaggtgtgagccactgcacctggccacaaagctttctttctaaagaggtgaactaaacatgaacaagccatcaagtacttcactgcggtcaagctgtactgatgtcaggtagcaggatttgtggagccaaccagttaaaacagcaaaataagctctatatgccaggtttctatgaactttcagaaggaaaaagaaaacacaggaccagaggcacctttttttgtttgtatgtttgttttgagatggagtcttgctctgttgccaggctggagtgcagcggtgcaatcttggctcactgcaacctccgcctcccaggttcaagtgattctcctgcctcagcctcccaagtagctgggactacaggcgtgtgccaccacacccagctaatttttgtatttttagtagagatggggtttcagcatgttggccaggatggtctccatctcttgacctcgtgatccgcccacctcggcctcccaaagtgcagggattacaggcgtgagccaccatgcccagcccagaggcaacttttaaaatgttggttttcaggaactacatgtctgctaaccttggacatgttgaaatgtaatgaatacaactattaaggttataagcgcaataaatatccttaaaaggggacatacaatcacagcaaaaatattttgctttttttttttttgagacggagtcttgctctgtcgcccaggctggagtgcagtggtgtgatcttggctcactgcaacctccgcctcctgggttcaagccattctcctgcctcggccttcccagtagctgggattacaggcacgtaccgccaagcccagctaatttttgtaattttagtagagacagggtttcaccatattgggcaggctggtctccaactcctgacctcgtgatccgcccgcctcagccgcccacccaaagtgctgggattacaggtgtgagctaccacgcccagccacattaatttgcttttaattagtagtaacaaattcttataatcagagtacaaatctgtactatctgtatacaattagtacttgatgtgtgcggggctgaagtatctcagaatagtatatcatagggcaaactaatgtaactggcaaaaatgcaaaaagaaatgaaatggctaatctctacaagaaatcacatgctgatctattttaaactgtaaaactttacatcatataaaaataaaattttcccatttataattacctgacactttcccatttccttgcctctcagtggaatacactacagtaaaatgtcatacattgagctccaataatttagaattgaaaacccagaggatggaatacagtttatcttttaaccacttacagaaaagaaatttcttaacaagcaaattcatgatgtaaaaatacaatgcaagtattttacctgcttaagggaatatacttttttcatgtacttttatttatttttatttttattttctgagatggagtttcactcttgttgcccaggctggagtgcaatggcgcgatcttggctcactgcaacctccgcctcccgagttcaagtgattctcctgcctcagcctcccgagtagctgggattacaggcatgtgccaccatgcccagctaatttttgtatgtttagtagagacggggtttcgccatgttggccaggctggtcacgaacccctgacctcaggtggtctgcctgcctcggcctcccaaattgctgggattacaggcgttagccactgcgcccagcccatgtacttttattttaaaagttaacataccaatatccataatcttgatcttggccagatgcagtggctcatggctgtaatcccagcactttgggaggctgatgtgggagaagcacttgagcttaggagttcaagaccagcctgggcagtatagtgacccccatctctaaagaaaaaaaccattagctgggcatggtggcgcatgtgagtagtcccagctacttcagaggctgaggtgggaggatagcctgagcccaggagtttgaagttatagtgaactatgatagtgccacaaaacaaaacaaataatcttgacctattcactaggaaactggactgtctatatataattgaacttaatattctataatcatgctttttgctgccttccaatttattcacattcataaattattactatttaaatttttaattagctgaagtactctattaatcagtctttatacctggctctccctagccacttaaactctgatttcttcattgatactcagggattcaatcaactttagaagtatgctagggaaaagatcagggtagcaaatcttccatataacaaattatgggggaaaagtttcatttcaaagtcaattcaatgaattttgaatcatttgctatttgttttccaggcctacaaaaatggtatcttaatcctaatgctgaaaaatgtgaccatttaagcagtttcaatgtgcttaaatttaaaaaaaaaaggcatgtaacaattatttatttgacaggtttccccaaaactgtagtcaggtaaaataaatccaatctgttatgttagtttgctactaaaggggaaaaaaaggatcaaacttacaggaaagccccacctcccctccacatgtagaaatctgtctaaagactgtctttaatgcccactatataaacaacattaaatattctaagttacaaaatagtgttaatggtttattggtaaaaatccaaactctagagtttatggaattcgtagtttggttggtatattaacactccatcttaatctttgctgctattacaaagaatgaggaaagctagaaatatctataaaaataaaataccttaaaaccgacaagcaaaatataaaagttgcatacaaattgccaataaatataaacatcacaatagaaaaattaatcttaacaaaaataaactcataattgctattaagacattataaaaacaaaaaagtttaatgtgcatgtatatttgcaaacagacacagtacactccaaacaatataattttactatcattattatataatgcagcatacaaggttactgaggtgtggtattttttgttgttgttgttgtttgcttttagtcttcttttctggaagaatgctcaccaaattcacaggaaagaagtgcctaggtgatcatttactgctatttactgcttcctggtatggagcaaaattgccctctggtaggtaactacatttctaattagtatgaaaggttctactattttcctttcttttgcttatttccccttaagcacaatttgcagaccctacttctatttaactgatcatacccttttaaatgccttgtcatcatttttcatagttcctgcatcctagaaaaaataaaaaatcatttaaaatattccttggtgtctagaaaagaaaatttctctaacaatagagattatcattttgctttctcacttaagctgatctgaatgatgatttggtactgcctttatgagcagtcctccttaataatgactaattagggccgggtgtggtggtgcatgcctgtaatcccagctacttgggaggctgaggcacgagaatcacttgaacccgggaggcggagtttgcagtaagctgagattgagccactgcactccagcctaggtgacagagcaagactttgtctcaaaaaaaaaaaaaaaaaaaaagattaattagaaaatgttgcctatgattccaggcaagttacatttccctttggacattggtactatacccataatcttgttaaaaagttaagtaggtttgctgttttatgtgcattatggatttcctccaacacagttgggaattaaaagaggtaattctactaaatattttgttttcaaatttacaaaataaatttggtgagcatttacctagatactttactgcataaaagctttccttggttcccttggacgagattcaagacaacaactaacattatttttatgaaactgtcacactcttggagttctaaaataatttatctttaaaattcttagcttcgtgctacttgaaaaataaaaatctacagcaccatcttctgaaaaggcactttctaagaaccgccttgctttaaaaaatgattaaaaaatttaactcaagagtctacgccctgacaaacgtctttgctttactgagaccctaacatagatacattagattctggttaccttagaaattagtctaaaaaaggaagggaccccgatggctggataggtgatttgacaggattctaattttgtcacaccatttacctgatacttcaacagggtttctcactggtaaatctcaaccctctatattgaatttaccatccttctatctttaattcaaattaaaatctttaacttccatattttaagaacaaaagattcttgagatttaatcaatgatgtaaacatctggagtactagttttgatgggtaaagtaatataaatttcaatgagtagtaggtaatattagcacaagccttgaccattataccttagtttaaaaaattatgttgactgacatggaaaattataaacttaaatgtaccattttaaaagtaggaaaaaagtcaaaataatttttccctttgtgtgtgtgtgtgagattatatatatacacactcatacatatacacacacacacactccccctccctgcttcctgggactcagcttggctttcactaatcacagtgtcatttctaacactgcaacggatcaagaatgttcttagtataagcaggacttttttaaaaagattttttggagaaaattctcactttctgatttctgtgctgactgacttacctactcttggctgattttttgactcctatagaatcacaaaagtgcttttctatgatcaaatatgaggactgaaataggaaaacaagagttctaaattagggttatactgctacacaggaaggcgttacttgatgtcaaacctcccaacaattcttactgaagctttaagacatttatgaattctcaaaaagaatgaaaataatgaatacttcatatggataaagccaaaataaagacgccacactaatgatatttttgcagcttgactaactaataaaaggtaatttaagtagcaagttactgttaagggcaacctgcctgttcaacagaagaacatctaagaggataagctaagcaaacatttaactcaggtttaatgatactgaatgaaaattttgcagagttgtcagttaaacttcttggtaaaaatattaaaatcaagtttgaaataggaagactgcaacatattctagctgtatcgaagtcgtttgcttcttgaatttcataaaaatcactgcccttggcaaattcatgtagggctctaaacagatccatcaagttccttgagtcacaaacggtctctaattcctggtctgcaatccatctaaatacttcggatccatcactggcatgcttagcgctcaccctttccttgaacacagagatccgctgccagtcattcctgctgaagggcaagtcaggttttatttccctagacatgccttcagtctttcatgactctgtcagaaggcctatcctcctaaaatccattagagaatacacaagcaaacactaggcagtggtgggctgtggagaagctagcttggaaactggtctagatctttagaaggctgagaatccctgtgctggaaagcagagatgcctctatcaagtgccttccaaaacactcagtaattcctactagaatccctgctagactctcttctaggaatagaaatatattaataggttataaacagggatttcccttagaatgatagtttttccaagaaacttgttagaagatcactattaagaaaaagaaagggaatctaatatttctgttgaaatgtgccaaaaaaccagtactgaagaggctgaggtaccctttttcaaactgtaaaagtcaaaatctacatttctaaaacaaagaatatcctgatattaaattgaaactaaaatggcagcaccctttgttactttgatattccgtgtccttactcttaggaaaaaaaagggtctaacactagccttgaatcctgcttatctccttactgtttagtgcagtaactgtcagaatctacttaaataaatatagcagctacaatattgtaagtgtatggtcctccatgccagtaacctgatactgtgatataatacatgtatcagcactttatgtagacacattaaccatcaagaatatacattaaactcccaactcttcttcatatgaaaatcaattatctagttgccagactgatattttacagtcagtctcgtaagatacatcacagaaaaaagaagaccaaaatctagcattcatgatatagttagtgagcaagggcaggagcagaagggtcactgtgaatttcatgtttaacttaaaaaaaaaaacttttttaaaataaaaaagattagaaattctacaccagaaatgcaacaataaataggacaaatttcaagaagcatttgtcacttagccttttatcttaaaattctaagcacaagttttcttgtaattaagaaccaatggtaattaatataccaatttgttagcaaaatagaaatatagtatacatactctttcaagttaatcaactttaaactagcaatgctgactagtgtaagagcactctaaaaaagaaatcactcaaaaggtaaagctttataatttagaaaaaatatttttcctcttaaaaaagtccttccaaatagatttaaattaagggctccactctagcatatatgagtgactgaaaattaggtgagagagtacatagagaaagggtatctacagtcattccctaaagtttcccacatgaatctgtgcagctcccatgataaaggaagatgttttactcacactgatcaagcatagacgaattaaatttttatcatcttgggtatactattttcttctcttgcccatgatcctgactatattcagtaaaatttcagtgtaaaaaaatccatctttataggaaatttttctggaggagatgggagaaggctgggagaaaaaatgtatatacgatacaaatattaccttttgtaaagttctttgcaacagtgttgtaaattgcatttcagacacttcaaaataataaacatacaaaatacagtactttcttagttttctggcagagggacaaaagatttcatgcctgtcagaggacatgggctcagattttaggctcaaaatacagtgaattggcaataatagtggattacaggtaagagagaaactaaagatctaaatccattaggtttcacgtgcagatggaattctgaaaggctaacaacaatgcccactggaaacaatctgtagtatctatactctgaaccagtgcaaaaaaaaaaaaaatcaaaatgcaattttcatgagttacaaagtgcaaagctcccctgaatccaatgttactgataaactcagttttgatagctttatagtactttttaataccttaaagtgtaatcaataaaagttttgtaaaacaatttcccacgtttcagtgatttaactgatttaaaatgatcaaagtcctaacttcctttgttactatcaccttaattttaaaaggaaagttatactggtgatacattagcaaaagttttaaaatatcatcttgcattttcctgattcattttagtaaatgaaaatgggcatctagccaatatgattcttcaataaacacaatctatttgcaaataatttaaatatgttaagctattcacaattatataaaagttcaactttatttctaatattcaagttggactcatttaggcaatttcacttcattttcattatgatttttttttcttttgagacggagttttggttttgttgcccaggctggagtgcaatggtgcagtcttggctcactgtaacttccgcctcctaggttcaagcaatcctgcctcagcctcccgagtagctgggattagaggtgcccactaccacgcccagctaatttttgtatttttagtagagacggggtttcaccacgttggccaggctggtctcaaactcctgagctccggtgatatacctgtctcagcctcccaaagtgctaggattacaggcatgagccaccgcgtccagccttttatcatgatgaattttaaaagatatgctttaaaactgaaaattacaaaactttccttctgaaattaaggctgtattctttgcccttttaaactatggaggtgcctgttcctcctactatccatggtaaagatgcagacacaactttcctttaaaactgcttattgcactaaaagatagcaaaaacaagttgtcagttcttaaaataaacatgattatatttctataaaagatgctgccaatacaattctataattattaaagcactattctaataaatataaaagaaaaggaagctatacttccaaacacatacatatgtgtttatatacacacacatacatatatatatataaaaaatatatgaaaatcacattaaggtatgagaggcagcaagtaaactatcaaaaaacaaaacaaaaaaatccctcaacaaactcttctctctactcaatttcagaggtctcaaccctacagagctctaatcttttaaaatatttaccctttataaaacctttaaagaatttccatgtataacccatagaaacagaaggcttcagaatacacatcacttaccagagagaaagttacaacttctgacaggttttatatttatagcagctttaacaaactcactaaagaaaaagaatagtaggccgggtgcggtggctcatgcctgtaatcccagcactttgggaggtcgaggcgggtggatcacaaggtcaagagatcgagaccatcctggccaacacggtgaaaccccgtctctactaaaaatacaaaaattagctgggtgtggtggcacatgcctgtaaacccagctactcgggaggctgaggcaggagaattgcttgaacccgagaggcggaagttgcagtgagccgagatctcgccactgcactccagcctggtgacagagcgaggctctgtctcattaaaaaaaaaaaagaaagaaaagaaaaagaaaaaagaaaaagaatagttcaggttgctactgcttatatacaaattgcgcaaatggtaaatgtatgttctgagtgggaggggagagacgcactctcacagaaagttattttatgtatatatatgtgtgtgtctgtgtctgtgtatgtatgtatacatatatatataaaattttgtttcttaagacagcaatatcaagagttgagaactcagaattgtgtatgagataggagtcaggagtagggtatgcaaaataaaagtagaattctagtttgccatattttatattcaaacgaaccagatacatcaacatttgaatgtcactggtaggactgggaaaaaaatgtaggtgatgaaggcaagggaaatagagaaataaaggcggtagtgggggtagaataaaagggaaagaaaattccccaatggaatgaactctaaaatatataacagacacatatatatctattatcaatccagatctagatatatatgcatatgaagtatggatgtatatattttaaaaatacacagacaccttttacaagaatatatgaatgcacattaattttttgcacacataattctgaaaaatcactttgattattcatgaaggtgtgtattttttaaaccatcatttactttttctttacttttttttgcaaagatagttgtgctgccaagcaacttgaggtaaaggcattaaaagggttagactacaagaaatgaaaacaaaacaattgcgatacttcctataggagaccgcacaaaaagcagttggctggtttcatattgcataatgatgctgtgttccttgatgaagtaaacaatcttccttgtattaacataaggatcagaccttggcccccacacagtgttggtttctgtatggctggaggtgtccttactcaattgacttcactggaaacatacgttgtatgtcaattcatctttcagtacttcctctcagagaatatacttggactatttaagcgaagtacattgtgcgtaaggtatcttggtgaatctgtacagccttggcaagagcttgtggatctcgcccattgctttgtcctgaaacgtgacttccttcagcactgtcatgttctttgtccacaagatgatatctggctctaaatgctaccaggtgagcataatacgctggtgcaggtatagaaacagatcgtgtacagcgtacgtaagtgtggcagagctggtaagttagcagctgaagttcatctgcagtaaagcagttatcatcccataaaacatgatagtgtgaaggacgactggtaccctgtattccagcatggctacagaggtaaaaatcgaactcatatgggtgtgtaatgtctgtatcaactgttgttccagctgggatattgccacttcttccaaccctttctgtcctatcagcacaaaataatcgagtgtgatgtctcttctgaactacaatgtaggttattccaggttgatagtctttctccaaactgatgcaggcttctcgaattgctagtagttcataatataatacctgcctaaactgcccctctgaaacaccatcccgataaaagatgatacgagtaggcttgaaccgagttgacttataaaattgaataagaagttcccggaccatggaggccaagtcctggatgatctcctgtcggggtctctgaactcttactgtggcacagtatctgcttgggtgtgcatccatactacctacaacagcagcaatagaaggcttctttccatcaccagcaggtggatgagtgacatcggctcccaaaaagatcactggttgctggaacacagaaggtctttgatgaggtacaagaatattattgatccctccgagtttaacatttatctttaggcacaagtttgacagagtttgaggagatgtttttattacattcttgacttgaacacattgtgtagccatacccaaaagtgtgtctcctacacgtttcacttccgcatacactggtgtcttccccggcaggatgacgataataagctgtaggccagaatatgtgttcttgagatgccggaacatgggctctacgctgtctgccccctgtgcatatttgcagaagcatggctggccctggatgggcatccctgcatccttagaaatcttacgcagctggtctgtgaaacccttcaatatttcttctctgcactgcctctgtgtggcaaaacaagcgatagcccacattttgatttcaactcctgtgtggaattgtttccctcgcatgtcccatactccatggctcggtgttgctactgtccgattccgtcctccatactggagcataggtgctggaagtacgcgtccagttacatgagccatttcatcccgaactttaaattgaaactcctgaacaaatggatctgtttcataatttgcacttcttaccaatctgctaatttcctcttgtctatctggtgcagatcttgctgttgccttgatcatagtggaagtctgattgtctgttagcttcttgatacatcgttgccctgccacaatattacagacttctagtggcaggtaggtgtgtttctgttcctgcccgacttgcagacagggaaggtgcgggtacttcagctgaagagtatacttttctctgaaatactgcgctactgttctctccacagtttggccgttttctaactgtaaaggaaaggtttgatgactggcaggcctccttgttacattacaaacacggtatttccgtctcattgttccacaatgagtcacttcaaccttcaaaccttttatctctttggtgaattttacccgatgagaatcagtcagaggtcttggttgctcatcaatattatgaatatcaagaacttcacacatgaactgaattacaggttgtgctttgtagaaggcagtggcagaaattcatggagggcagatgtcgtagcaccacatcaacggcatggacagggttagtgctgattggcttgtctaattccagtggctcaggcaaggtccgtcctgtcagtacttcatgcagtaggtgccaactcacccgagagacaaatttgattgacaccttgaaaggtcgatcttttccaccttccccaggtaaagtaacgtctaaatctacctgttcactctcctaggacacttgtctggtttaatatctacctcatagaggtagacatcaatctttgggatttcaacttgaaaacagttagccagcagtttaatgggtttgcccatggtgccatagccaggtcttctgggcaccatgagtaggggctgggccccagcgggtcctgcggagccgatttccattcatggagctggggggagtgcttcgagggagaacggagcccgccactggcggcaaggaggcggcccggggggcgacgcggcgcgacgcgacgggcactctcactcggccccgaggcgggggcggcgacggcttcccctgagcaaccgcactccgaaagctctgggccggaagagtcgcggacggaaaacggcacaggactaggcgagaggaaggggagatgtgaggcgcggacagaggggagtcccgtccggaagttgcatcgcccgcggccgccgacgctcccaccgctcctccacgactgcgggccgccgccgccgacct

SEQ ID NO: 14027 - RNA, 3835 nt, Homo sapiens
  source 1..3835: mol_type = other RNA
gctgggattacaggcatgagccaccgcaccccgcctgttccctgaccttttaaacgaattcacgtattaacggagaatcaacatctaaatagacttttatttttattttacttgtttggacagaaaagaaaattcatcagctttcattagagtctccttaagtgttggaaacacattaaactcagaaatagtggaccttgtagaaaagcatcacaaattaaaaatatatttctccatgtggtaaaagtgctttcaatcccattaaagggcacagcaagggtgtttggaaacacgatctgaaatttggcctgcaatccgtggcatcgattccaaccacagggcgggggagtcaccatgatctagagcacaggagccacgtggggcccggagcatgcggacagcaacactcgcaataactgagtgaggacgaggcccatagcctgagtagaatagattctgtatttgtaaaaaatgaggtggttacatcaactgggttgaagggggactgggtaatcccagaaattccttgtttctggtctgtggggatggtcagatctgcccaccactctggcaccgaggcttccctggagacgcataaacctgggttgggaaagtgcccagatctgcctgggggacacacgagcctcgctgccagtgccgggcacgcagcctctccagtcctgccgtcagcaaccgcctccggccctcatgtcaaatcacacctgaccagagttgtcaccacagtcctgttttggggtttttccaaggccagccctgttgttctgaggggccactctgagcaggcaaacactgccagggtcactcactacacacagaggaaagacaatgagcaaatggccatcgtagagaattcggttgtgtgtttcagcaatgctacttatttttcaagacaagtaattctgccaatgatgacatctgcgacaaagcttagggcccgcgggctccccatgcgcctcgtggagagcaaccacgtctgttcggaagccagcggcccttcccggccctgccacaggccagaacacagaactgtgatcatgcaaagagccgtgactgaggccggggtcagcgtcgggggtggagaggaggggacatctgccttttacattagatctgaagcaacagtaagaaaataacctgaagatatatttaaaaataaaaaatagcatcatccttcactccaagtttttggcatttccctctctcccctgcccaccagctaagcagagggaatgagcaggaatgcctcgtttttcagaatgggcacccactccccatttcaccactgtacacccaggatgtgtgtcttcttctaagagaccggttcaaaggtgctggcatgaggcaaatgctggaaaaccctccggcctcccctgacacctgagccattgtaaccatgcagggcgtctttgcttccttcaagtcttgaacttgaaccacgtcccagattgctgtagatctttaggaagcaggcatctctcttagagcgtgctccagctcattctaccacgggggccttccttcacagtcaccagtccacgctgcctcgcaagctccacggatgtcatgagagaatctgcccttgagaacgtgggtgtaagtgctcatcacaccggcggcactgtttctcgagggaggacatgctcttcttggaatgcaaatgaggacagcaaccgtcctctgaccaggtccatcctgtccctccagaggccctgtgcatccctcccaggcagcaagccacacaccaggccgtgtccgggtctctgatgggcaagttggaacggcaggctctcctcctcctcttgcccctcccttgaccgagtcctgcgcccccagcatcagtgggtcggagaggcatcctccaagcccagcagctctctgacgagtctctctccaaactgcgcccggctgtacctcttcacgtggtaggcgtctgacattttgtacaggatgtaggcattgttgatggcgatgctgatggcgaaccagaacacctgctgccaggtcttgtttggtttatgagaaatgaaatacttgctgtatttgtcatcgtatctgcagatgtagctcaggtgagcggcaaacgcctccacggccaaggggcatgggatctccccactcttccttttgatgatgactccctgctgcaccggggagtaggcgttggtcaggaagcggaagtgtcctttgttgtaccagcagatcaaggacatgttccccttcatcttgatttggtactggccccgggccgggggtgtggctgggttggtcagcatggacagtgggaggccggtgcagtcactcttccgcgcgcggagcaagccgcagcagtaaatcccttgcttctcaaactcttcaaacagcgtcaggctggtgatgctgggccccgtgaaaatgatgtagttcttgcctgccgcgttccggcacaggctcctggccaccatgctgtggagctggggcttattcttcagcgcatccaggccatctgggcccccaccttccttcaggtggacataaatctggatgatgaagccagtggaagaacattgtctgacccagaggctgaatttccgctttttcctctttcgcagctcccgctctgtgcacgtggcaatgaatacaggatcctcatcgatcaggggttcatgtagcacctgggtttgggaaggcctgaaggcagagtcgaagctgttctgcagggagtcgaggaagggctggaccttgtagagcccgtgcgtggtctggctggagcggaaggccacgacgtggaagtacttgaggatcttctcgaagcgggcctggctcatgacgagggcgaggctgcggttgctgtagaagcctccgctccagatgctgaggacggactcgcagtgggagatgctggtggagatcatgtagcccaggaacgccttcatctccgtcagcgtcacctccacccaggctccgtcgctcccaaaccgctcctggaacttcttggcatacatgtttgtctgcaccaccatgttcttgaggacgttgtctgggacaaagagctggaagaagtccacggcactggcgctggggggcatctttcgggtgggaccgccggtatcctcgaagcgcgggggcgggcggtcccgcagcgctgcgctccagcccgcgccggcctcgtcctcctccggctcctgtgcgtccggggcgcggggcggtggcggggcggcccctgggggtcccgggggctcgcgctcgtcgtccgaggaggcggccgaggaggagcgcgaggcggccgaggtgctgtagaaggggttcccgccgctgtccgggccggactcgccgaacacgtcgtccgagatgtgcaggctctcgtagcgcgcgcgggcagcctcgagcagcgccggcgccctcctccgcgcgcccccgccgccctcggccatggccccggccgccgcccgcgcgcccgcccccacagtgcctcccagccgcacacgccgggccctgggcccgcgccgcggcccgccgccccccaccagcgcagcccgcagcacagcgcccgccgccccgtgcccggccggcccgccgtcttggccgcctcgggcccagcgcccggggaagcgccctcggagctcgggcgccgcaggctgcgggccgcggcgggaggcgagccgcgcgcggggctggcaggggcgacccagagcgggcgggacgcagaggctgcggccgagaccaggcgccgccgccgccaccgccgccaccaccgccaccaccgccgccgctgcgtctcctcggcgcccgccgcctccctgcccgccctctccacggcctccggcgctcggctgcc

SEQ ID NO: 14028 - RNA, 2422 nt, Homo sapiens
  source 1..2422: mol_type = other RNA
gctgggattacaggcatgagccaccgcacccggccaacctgtggcacttttaaaatagatgccttacactcaggaatctagctaaaagctcaaacctatgcatattcatggtggtgttggaggttgaatcaactgtagtgacgtgaatcatctcttttctcccatttactcaatgattagctttcttcttatggtgtaaggcatttatcattggcgtattaaatagtgtataagacacccaaatctaatgttaacccaatactttaatatgaacgttatgatcagtaggtagtatcttagatgatacatttaatcacagacaaaacaaaaacctatctgtatatgatattaagaggagcacagaattggataaagtagggtttatcttagtcggagaccaaatggttttgatatgtggttcctagaccagcagcatcagtagcaactggaaatgtgagatgaacattctgaaacacacatctggtcaagaaccactgttttaatagctttaaccacaaaacatccacattgttccctaaagttatgctaagagtaaaacgagtaactggttaactgcccatgatacatcaatttaatggaaaattatgcaactgtcaacaagaataagcatatctatatgtattgatataaaacaatctctaatatagtgttaagtgaaataagcaatatgcagaacttaaaaatactttttagccgggcacggtggctcacgcctgtaatcccagcactgggaagccaaggcaggcagactgcttgagcccaggagttcaagaccaacctgaatgacatggtgagaccctgtctctatgaaaaacacaaaaactagctgggcattggtggtgtgcgcctgtaatcctagctactcaggaggctgagatgggaggatcacttgggcccgggaggcggaggttgcagtgagccaagattacgccacagcactccagcctgggctagagtgagaccctgtctctaaataaataaataaatctaaaaaatttaaagggggcatgtgtctgtatgtatgtatactttacacagtaacagaatatctcttaaaaaacataagaaattagtagctgaagtttcctccaggaagggaagcaggaagcagatgactggattatagggatggaagaaacatttttccttctttttttgagacggagtctcactctgttgccaggctggagtacagtggcgcgatctaggctcactgcaacctctgcctcccgggttcgaccgattctcctgtctcagcctccccagtagctgggactaggggtgcgtgccaccacgcccagctaatttttgtatttttagtagagacggggttttaccatgttggtcaggatggtctcgctctcttgacctcgtgatccgcccgcctcggcctcccaaagtgctgggattacaggtatgagccaccacacccagctctggaagaaatatttttcactacatgtttttgtactgtttgcatgttacattaagtgcatgtattattaattcaggttaattaatttaaaaatttaagtttaagggcaaaaagaaccactactttagagagaatggagatactagcaagtaaaatatatgaaagagctagttggaaaggaagccaagcatggagtagaacgtggggccgtcagctgctaaagggtactgagcgttaatggagggcggagcaggaagaaaagtcagacctggcaaaaagatcatcttccctccatatcctttctgaggtaatattaggtaaactgagacctggaccagagggctcaattatatccatagtcacctttattctgaattaaccatttatcaagagtgcgcctgaaaagagtagaaaaaaataaaggagcccatcaaaaaaaagttccctggcaagtgggagggaggacatgatgttaggagccctgtttggggaaggaaatgttatccaggtcatggatgccatttttgtcaatgattcgaacactgaaggttggcagattcaggatgaagcgtttctggagctcctccagacatttcctaaggagttccactgccctctcacgtgagatagtcggtgtgtagtatcggtcgaggatactgagagtcaggaaggcaccatagccgtgggctgcaaaaggggccttggccaaggctgccaggtagtccatgtaatacagcgctggcccttcatgctcatcatagccagccaggaggaggttcacatgatatggggtccgactccgaagacagtcagccaggtttcggcgtgtgaagttagctgctgccgtgggagacaattcatatccatcttttgtacactcagagtaaacaaagcatagactgaggggtacaatcctactctagtccctttcctcatgcaacagctatgaaatagctggttagtact

SEQ ID NO: 14029 - RNA, 2553 nt, Homo sapiens
  source 1..2553: mol_type = other RNA
gctgggattacaggcatgagccaccgcacccggccaacctgtggcacttttaaaatagatgccttacactcaggaatctagctaaaagctcaaacctatgcatattcatggtggtgttggaggttgaatcaactgtagtgacgtgaatcatctcttttctcccatttactcaatgattagctttcttcttatggtgtaaggcatttatcattggcgtattaaatagtgtataagacacccaaatctaatgttaacccaatactttaatatgaacgttatgatcagtaggtagtatcttagatgatacatttaatcacagacaaaacaaaaacctatctgtatatgatattaagaggagcacagaattggataaagtagggtttatcttagtcggagaccaaatggttttgatatgtggttcctagaccagcagcatcagtagcaactggaaatgtgagatgaacattctgaaacacacatctggtcaagaaccactgttttaatagctttaaccacaaaacatccacattgttccctaaagttatgctaagagtaaaacgagtaactggttaactgcccatgatacatcaatttaatggaaaattatgcaactgtcaacaagaataagcatatctatatgtattgatataaaacaatctctaatatagtgttaagtgaaataagcaatatgcagaacttaaaaatactttttagccgggcacggtggctcacgcctgtaatcccagcactgggaagccaaggcaggcagactgcttgagcccaggagttcaagaccaacctgaatgacatggtgagaccctgtctctatgaaaaacacaaaaactagctgggcattggtggtgtgcgcctgtaatcctagctactcaggaggctgagatgggaggatcacttgggcccgggaggcggaggttgcagtgagccaagattacgccacagcactccagcctgggctagagtgagaccctgtctctaaataaataaataaatctaaaaaatttaaagggggcatgtgtctgtatgtatgtatactttacacagtaacagaatatctcttaaaaaacataagaaattagtagctgaagtttcctccaggaagggaagcaggaagcagatgactggattatagggatggaagaaacatttttccttctttttttgagacggagtctcactctgttgccaggctggagtacagtggcgcgatctaggctcactgcaacctctgcctcccgggttcgaccgattctcctgtctcagcctccccagtagctgggactaggggtgcgtgccaccacgcccagctaatttttgtatttttagtagagacggggttttaccatgttggtcaggatggtctcgctctcttgacctcgtgatccgcccgcctcggcctcccaaagtgctgggattacaggtatgagccaccacacccagctctggaagaaatatttttcactacatgtttttgtactgtttgcatgttacattaagtgcatgtattattaattcaggttaattaatttaaaaatttaagtttaagggcaaaaagaaccactactttagagagaatggagatactagcaagtaaaatatatgaaagagctagttggaaaggaagccaagcatggagtagaacgtggggccgtcagctgctaaagggtactgagcgttaatggagggcggagcaggaagaaaagtcagacctggcaaaaagatcatcttccctccatatcctttctgaggtaatattaggtaaactgagacctggaccagagggctcaattatatccatagtcacctttattctgaattaaccatttatcaagagtgcgcctgaaaagagtagaaaaaaataaaggagcccatcaaaaaaaagttccctggcaagtgggagggaggacatgatgttaggagccctgtttggggaaggaaatgttatccaggtcatggatgccatttttgtcaatgattcgaacactgaaggttggcagattcaggatgaagcgtttctggagctcctccagacatttcctaaggagttccactgccctctcacgtgagatagtcggtgtgtagtatcggtcgaggatactgagagtcaggaaggcaccatagccgtgggctgcaaaaggggccttggccaaggctgccaggtagtccatgtaatacagcgctggcccttcatgctcatcatagccagccaggaggaggttcacatgatatggggtccgactccgaagacagtcagccaggtttcggcgtgtgaagttagctgctgccgtgggagacaattcatatccatttcgcatcttataaagttgcacgtttttctgaatatattctgcaaactgtacagtgtctccagcctctccaacacacaggagtaatatcttttcactcatcttaaacatcttgtcatgatcgatgaggtactccatggtggcggaaggccaggggctgcaggtccgacacagcacgagactcgcccgcttccaggtctcaccggtgagacagcacctcagagcgaagatt

SEQ ID NO: 14030 - RNA, 2628 nt, Homo sapiens
  source 1..2628: mol_type = other RNA
gctgggattacaggcatgagccaccgcacccggccaacctgtggcacttttaaaatagatgccttacactcaggaatctagctaaaagctcaaacctatgcatattcatggtggtgttggaggttgaatcaactgtagtgacgtgaatcatctcttttctcccatttactcaatgattagctttcttcttatggtgtaaggcatttatcattggcgtattaaatagtgtataagacacccaaatctaatgttaacccaatactttaatatgaacgttatgatcagtaggtagtatcttagatgatacatttaatcacagacaaaacaaaaacctatctgtatatgatattaagaggagcacagaattggataaagtagggtttatcttagtcggagaccaaatggttttgatatgtggttcctagaccagcagcatcagtagcaactggaaatgtgagatgaacattctgaaacacacatctggtcaagaaccactgttttaatagctttaaccacaaaacatccacattgttccctaaagttatgctaagagtaaaacgagtaactggttaactgcccatgatacatcaatttaatggaaaattatgcaactgtcaacaagaataagcatatctatatgtattgatataaaacaatctctaatatagtgttaagtgaaataagcaatatgcagaacttaaaaatactttttagccgggcacggtggctcacgcctgtaatcccagcactgggaagccaaggcaggcagactgcttgagcccaggagttcaagaccaacctgaatgacatggtgagaccctgtctctatgaaaaacacaaaaactagctgggcattggtggtgtgcgcctgtaatcctagctactcaggaggctgagatgggaggatcacttgggcccgggaggcggaggttgcagtgagccaagattacgccacagcactccagcctgggctagagtgagaccctgtctctaaataaataaataaatctaaaaaatttaaagggggcatgtgtctgtatgtatgtatactttacacagtaacagaatatctcttaaaaaacataagaaattagtagctgaagtttcctccaggaagggaagcaggaagcagatgactggattatagggatggaagaaacatttttccttctttttttgagacggagtctcactctgttgccaggctggagtacagtggcgcgatctaggctcactgcaacctctgcctcccgggttcgaccgattctcctgtctcagcctccccagtagctgggactaggggtgcgtgccaccacgcccagctaatttttgtatttttagtagagacggggttttaccatgttggtcaggatggtctcgctctcttgacctcgtgatccgcccgcctcggcctcccaaagtgctgggattacaggtatgagccaccacacccagctctggaagaaatatttttcactacatgtttttgtactgtttgcatgttacattaagtgcatgtattattaattcaggttaattaatttaaaaatttaagtttaagggcaaaaagaaccactactttagagagaatggagatactagcaagtaaaatatatgaaagagctagttggaaaggaagccaagcatggagtagaacgtggggccgtcagctgctaaagggtactgagcgttaatggagggcggagcaggaagaaaagtcagacctggcaaaaagatcatcttccctccatatcctttctgaggtaatattaggtaaactgagacctggaccagagggctcaattatatccatagtcacctttattctgaattaaccatttatcaagagtgcgcctgaaaagagtagaaaaaaataaaggagcccatcaaaaaaaagttccctggcaagtgggagggaggacatgatgttaggagccctgtttggggaaggaaatgttatccaggtcatggatgccatttttgtcaatgattcgaacactgaaggttggcagattcaggatgaagcgtttctggagctcctccagacatttcctaaggagttccactgccctctcacgtgagatagtcggtgtgtagtatcggtcgaggatactgagagtcaggaaggcaccatagccgtgggctgcaaaaggggccttggccaaggctgccaggtagtccatgtaatacagcgctggcccttcatgctcatcatagccagccaggaggaggttcacatgatatggggtccgactccgaagacagtcagccaggtttcggcgtgtgaagttagctgctgccgtgggagacaattcatatccatttcgcatcttataaagttgcacgtttttctgaatatattctgcaaactgtacagtgtctccagcctctccaacacacaggagtaatatcttttcactcatcttaaacatcttgtcatgatcgtccttcatctggacaatattgctggcggccacccggtcggaggcgacaagaacatagtcggggccttggataccgatgaggtactccatggtggcggaaggccaggggctgcaggtccgacacagcacgagactcgcccgcttccaggtctcaccggtgagacagcacctcagagcgaagatt

SEQ ID NO: 14031 - RNA, 1541 nt, Homo sapiens
  source 1..1541: mol_type = other RNA
gctgggattacaggcatgagccaccgcacccggccaatttgtttcatattctatgttaagccctcacatttatctaccttgccccctgctttagcttgcaacagtcaaatcaccttgagggccctgaccaggaccaaaataataactcgaatttgacggaattgtgcaaggagtttgagagacctcagcacccggcagatcctcagaagctgaagccacaccgattggcctgttacccctaccaataccacaacctcgggaagcagggactgtggaaaacacacaggttataagtaaaatacaccccaaggcacccaggcagaattgcagcttcttcatcttatcctcttcattgttccctgggcgttatcctttgaatagcattctctgagaagtgcttactattcagcctttctatattaagttgcttaaacactatacttcaacttgttcagatataaaaagggggataaaattcatggttatttaattaggttgttgtggagcataaatgagataatgtaaggaaaacacttaaaatagtgcttggcacttagtaagtgctcagtaaccggcagatgctcttgttggcattgatgttgtagttagtctactttgctcctaataccaacaactcctgcaatgattgatgtttagttttaggaaaaaaaaatcaaaagaaagaagttaagtaaatttttgtttcttcctattatcatgttaacttgttctttcgattcacctaggcacattcttcatcccactaaacgaaccctcaggatctctatccttaccaacatggtaacaacaaagtcaaagacattccaggcactcttccagaaaacagaaaagttggatagccacttaagaaggatctccaggatgaaaataagcaagataaaccaagctgccccctccaaggtcagcttcaatggccatagtttggtatttgtggattccagcaattactcaaggacccatccggcccacaaagaaagaggtggcctctgactgcagcgcacatgaagcctgctcaacagcctctgggcatgtgaaatctgttctatacgttgaggctttatagagacgcccactagctggtgttgatctcccaacataagtttcttctggcgggaaggatcaagtaactcctgatagtgtgtcgcagcacagcttggctcaagccttgcaaatgctcgatgagagagaaagtatcgatgagacgtgaacgaatggcatcagctcggggaagctgcatctgcccttcttgttggtaagcggccatgtctgctcagcccaggttctcttcgcccactcagtcctgacttcacgcttccacctccagctcaggcgccccctgagcccggctacccctacgcaggacgagctcagggccggctcccagcctcactgcgccccatttcccgccccgcccgacccccaggtttcggctcaccccgggacccggccctagcccctgcccccagcccaggaccgggcccagccacgctcgcccagacactcgccgcctcggccccgcc

SEQ ID NO: 14032 - RNA, 4743 nt, Homo sapiens
  source 1..4743: mol_type = other RNA
gctgggattacaggcatgagccaccgcacccggccagacagtgactttgatgggtggtagaggcagaagtgataaacggtagtgaattctataaatctggaggtagaggctgacaggtggaacaagggaaggagggagacagaggtagagagggaagaggaaggaaaggagaaggagagaaaaaaagaatggcaacaggattctgtctcagaaactggaaaggtgaagtcaccaataaactaaaatgaggaagactacaggaagaacagacaggagaggaaaattcatagttgagctttggacaagtttgaaatgatttattacacctccaagaagaaatataaagtggttggacagaaatgaggaattcagggcaaggtccaggctggagatataaaaatgtgagagtcacagtgcagagatgatatatcaagccttgaatttggatgaaacaaagggccatccaactgtgagagattgcagcaatgagtaaaaaccaagaaggatgtaaggcagagaagaaggcttgtgaatggtactgccagagacagacatttaaaagacaaaattttaatatttttaatagacaaccagtaggagtgtaagcataccaacctgctcccccaagaaattcctctacaactgcaaggccaattgcagctccttgtctgcttcattgaaagctaaacctgcctgcagaaaagctcagcccacagcacaattctaggtaagcctctgcactacctttccttaaactaggaaccactatctgcagatgtttttgaaaaaaattccataatcgaaagagcaagaaaaaaagcataaaatctgactctgactccattaattagaagacaagagtgaattccttgaaaagaaaaaaaaaatccctttaattaggatcttcagacagttgagatgattctgtatccacaaagtaagatactatgaaaaatagaacaagaaaaagtttgtggaaattaaaaaatatgcttgcctacatttttaaaatgttcagtaaggagactaaagatcaagtcaagcaagtattcaagagtagaccaacaagatcaagtcaaaaatcaagagagaaaaaatatacaactgacagattaaagtaagggcttatcatccaactaacagaatttccaccagagaacaatgaaaacaaggacagcaaattttaaaacaaataatgcaagagtatttcccacacggaagagaatgaattttcaaattaaaagggtacctaatgtacctaactagcatctagacataccacagtgaaatttcagacaccaggaacatagaaaaaaaaaagttcccggagaaaaaaatcccaggtattacacaatggaataagatgggcaaccaagttctcagcatcaacactgaagcctcaagataatgaaactatgccttcaaagttctgaagaaaatgacttcaacctataattctgtacctagtcaaagtatcaaacaagtacaaggatagcttcagatttccaagaactcagaaaatttaccttctatactttcttaaggagtttctttgtgacgtgattacaaaacggagaaatgcactgagaagacaaaatggaattcaggaattgcagagccgactcaggggaggagggcgcctcgggatgatggccttgagcaggcctagagcaagcagtgaggtcagaaaaggaggagagaggctccaggaggaaggtacctaagaaaaagtgggaaacccaaagatttcaaagcacagagtgataagacttttaggctacagtacaggtaggcaatgaaagaagggaaaaaagaagaacctaagggaaacaaaaaagggggaaaaattaaaaaaactctagagagttcccacacaaaactgtacaagaaacagaatgtaaatttggccttgtaatatttatatagtctttaaaattttttttttatttttagagacagggtcttggtctgtcacccaggctggcacaatcacagctcactgtaacctcgaactcctgggctcaagcaattctccagagtagccatgactataggtgcacatcatcacacccagctaattaaaaaacattaaaatatatatatagatgagggtctcgctatgttgcccacgctggcctcaaattcctaggctcaagcaaatctcccacctcagcctcctaaagtgctgggattacaggtgtgagccaccaaccatgcccagactaaatagtcttaacagtgtaaatgcttactgtttctcaacttagagtcaatcgactaagtcttaactaaagtagggaacaaaatgtaaatttgatcagctttgacaatataaaagaacaggtgacaatttagaaggtggaggcaggacagaatgtaggtggcggcaagaaagaaaatataagacttgaaagagaggcctggcatggtggcttatgcctgtaatcccagcactttgggaggacaaggtgggcagactgcctgagctcaggagtttgagaccagcctgggcatgatggtgagaccctgtctctactaaaaattttattaaaaattccaggtgtggcagggtgtgcctgtagtcccaagctactaaggaggctgaggcaggagaatcacttaaacccaggaggcagaggttgcagtgagccaggattacgccactgcactccagcctgggtgacaaaagtgagactctacctccaaaaaaaaaaaggaattgaaggatacatatctttcagaagtcaaaatatactgaaatataaccagacaagaaatatttaagttactacttaaaattactaaagtaaccaataaatgaattaaaaattgattttgctgtatgagcttggaagcaagggaaaagtataaatgggctagaacctgacatacagcaagaaatcaacaggtactatctagttggtcaatgaagaaacagtataaagcatattattacaacacggagaaagaaacagaagcatttaaaagtgggggattctgcggagtgggactagtatagagaagaatgaagtaaggaatgttgctttttatttttaatcttttttatactatttgattattttctcatctatcaggagatattacattgatatgctttctttttccagattttctatggtgagcatgtatttcataatgcattttatttcaaatatatgggatgcttccatacattataccaaacaggaaaaataaaaggaaatccacgcctagacacatcgtagtgaaactgcagaacatcaaacacaaagagaagatcttgaaagcagccagagagaaaggacagatcaccttgatttttttctacagaatctccttttgtttcctcttctttaatggggggacttattctgggggtcctactttgtccctggaccacttctgctagcaattcttcttgagaagttcgagttctgggagcaactggaagtgtctgtttctgtggaactgtagagtagttagttgtttttgttacggattcttgagcttcagatatagccttcaaaatcagattcttgttagcttgtttagaaggtggaagagaaggtctcctttcaggctttgcaggcacagacacactgctggagatgcttcctgttcgagacccgtaatcatcatcttcttcctcctcttctccatcatgattgaatttttttactttaacaactgaacttaccacaggcaactttctcttccgaaagttttcatcctccatactcattttctccgagttgtttctaaagaacggactatacgtttcttctaagctgttaagcacctctggttcacacaaacgtcctgtttcatatacccaactactctgcatatcaagctgcttggcagcatgaatactattctgctgctgttgaaattgcaacctgtttaaatgaacaccactatctgcatttctacttgcaggtggtcgataaatttcaatagaagggcgagaagaaccatatgtaagtgtcactgtaggttttttctgagataagggattctcctgcacaaagttgaggtcttcgtcaatgagatcatctggttctggcttaatatcaatcacatcttcagagggtgctggctccctcaaaggtttcactgttgacattagtcgggttgcagctccatcatcgtaagtctgtctgacatttgtggtttttgactcctgcgaacttgtagaaactctggaatctcttttttcaggtctcgcgctaggaatggcaagtggtggcactgcagcttcatgcctcctctcatctccccgactgaaattgctcttgtttgaaggcacgttactatcaaagatgttggtatcagaagacttcagactagagggttcagttgtaacagagcgaagtttatctaatacaccatgaagccatacggtgaatcgaattgtgttgttccctagaaacagggacagatcctctgtcatttggtcctgacttttcttgttggccaccatcaccataatgtaatcaggaagttcttcatcaacataagctcctaattcttgtaatttccccttaatggcactccggatcttgcggctgatctcggtgccgatctccatggctctgcggcgtgcgggaactcagcactgcgcggcgcttggcttacccggaggctgccgcggactcctaccccgcagccgggacaccaccgcctcctcctccgttccgcccccggccgcgcacacggcgtatccccgccccggccggcact

SEQ ID NO: 14033 - RNA, 6130 nt, Homo sapiens
  source 1..6130: mol_type = other RNA
gctgggattacaggcatgagccaccgcacccggccatagattttttagtgagttagaaatgaatgtaaatttccttttataggagttagacatttatttttaacaattaaccactgaattcattttcagaaataggcctgaattgcttgttaatttcattacaggaagtaactctaaaagccaattccacttccaaactataattaccatcatctgaatttaacagggaaagacatcttccaagacttcttttgggcggatgcttagttttagaatagccaactttaccctaacccatgtacaagacagttctccaggtggccttggactgacccagttctcccttcttccttgcttgtagttcttaagaataactgtagaatgcactgggaatgcaatatcctgatatggaggaactgcctgaaacaggttggccttgttgttgtccctcctagggaatgtaacatcttgatttagggaactgtttgagacagcgaggttgtgttcctctttcccctggaaggaggatgtactttaaagctttgcccaatgagttatgtggctcctatggtatataacccaaggcaggctgtggtgcaagtggggcacgtacaatcaagactccatcagccccgccctgggcagctttcttgagccctgggggactggctcacaatggagccagggcctcttttgtcccttgcttcctgtctgtaagtaataaatctgcttcatgtaatgtattgggtgtgagtgtgttctgtcacaatggaatcagacaggttggtaaccagtgtacactgaacctgcttggcaccatgtagccctgggaaaggagaaaggcggtcacagcttgccctatatggtgatgccagcacactgtgcactgtactgtgcaacagaaaaaggtgcactgaggaggatcggctgcttcttcccattgttgcttctttagtaaatcccctatgagtttttagtcgctttctaatctacaagttaaaggatatctcattaattttacagatatatacatatactgtaacaataggaaggaagtctttcaccaaccactaatactgtaaagaaagcattgtatcgatctagtattatttaatgaagacggacagcaattttaatacaatcttcttttccaagacctttgacagaccttaggcccattttccacctttatgtctaggaaagtataagtaaaacacttttgagggcataaaaaacacaagcttcttgttaaggtgtatcagtagccagggaaatctgctgtgcccctttgagggtcatctaactaaggcatggagaaagaaactgcctcaagtcagtttctatcacctctgcagggaagctggccatgcaaaccaggacatggttcaaagtgaaaaagagtgtggttaataatcatgccagaacaccaggtataagatgtaagggcaagtcaggcattctgtacattgcttctcccttcagtttggaaaactcactgcagtagggttttgacttatcgtttcacaagacagctaggaaggccaggcacagtggctcacacctgtaatcccagcactttgggaggccaagacgggtggatcacgaggtcagatcgagaccatcctggttaacacggtgaaaccctgtctctacttaaaatacaaaaaatagccgggtgtggtggcgggcgcctgtagtcccagctactcaggaggctgaggcaggagaatggcgtgaacccgggaggcggagcttgcagtgagccgagatcgcgccactgcactccagcccgggtgacagcgcgactctgtctcaaaaaaataaaaaaaataaaaaaaaataaaaaacaagacagctaggaggaaagcctgtatgctttggaaaatgcatatcttgtgtgtttacccttttaaaggtaactatactttgaaacaggtgaactgcagaaagttaacaaagacttctttttttaccatgtttacctttctaagaattctatgcatttcctagggcatacatgcaaaagccttcacatttccccctttttaaaagagatatttctcaaacttatacgtatacagttcagtagtgttaagtacaatcacacttgttttgcaacagatctctagaattcttgcaacacaagctctgtacccactaaatacaaattcaccctctccccttcccccaaccgttgcttggcaaccacctttctactttctattgtatgattttgactactttgcatacttcacatggaggaatcatatagcatttgttcttttgttggctggcttatttcacttggcataatgccttcaaggttcatccacattgtacatttgacaggatttccttctttttaaaggctgaataatattccattgactgtatataccacatttcctttatctattcatctgttgatggacatttgggatgcttccagaacctcttggctattgtgaataatgctgctatgaacatgggtgtacaaatatctctttgagatcccgctttggtggtaattcttatggtaattctgttttcagttatttgggaaacctgtgtactgttttccgtaatgactgcaccgttttacattaccaccaacagtgcacaagggtttcaacttctctgcatcctccccaatacttgttatttttttgttcttctgatagtggccatcatgatgggcgtgagacgatatctcattgtggttttgatttgcatttccctaataattggcaatgttgagcatattttcatgttcttattggccaattgtataacttctttggagaaatgtctgtgcaagtcctttgcccatttttaaaaattgagttatttggttttttgttgttgagttgtagaagttcctcatatattctggatttgggctccttataagatagacgatttgcaattattttctctcattctagagcttgcgttttcactttgttgattgcttcctttgacacacagacatttttaagtttgatgtagtcccgtttccttcctaacgatctttaagtgtacagttcagtagtgttaagtatattcatccaaccctatcttgcagaccagatgacaaacatattaatgaaagaaatactaccagtcattgacgcaacagagtctgaacataggcttagaggcattcagaaacattccaagatatttataagcaagagccacaggagcatgaattcctcagaatatgtagaattatctagattttagcctatctgacaagtttctctccctattaccataacaaaagtcttttaaaccactgtataaactgagatatttaagttaatcacctgccttgcaaagaaccttgactaatgagtaaataaagttcagacagttgtaaagggaagacgggatagctctttcactgtagaaaacattatcattatatactatgtaacagcgtgcaaataatacaaaataataatataaactataggctattagattactagtcctttgaaaaatatttctggaaggccgggcacggtggctcacgcctgtaatcccagcactttgggaggccaaggcgggtggatcacctgaggtcaggagttcaagaccagcctggccaacatagtgaaaccccatctctactaaaaatacaaaaattagctgggcgtggtggcatgtgcctgtagtcccagttactcaggaggctgaggcaggagaatcgcttaaacccgggaggtggaggttgcagtgagccaagatagtgccactgcactccagcctgggggacagagcgagactccatctcaaaaaaaaaaaaaaaaaagaaaagaaaaatatttctggaaatgtgcaatgaaagaattctaagttctaggcactttaagcattttttcttttcttttctttttttttttttattagacacagagtctcactctgttgcccaggctggagtgcagtggtgtgatcttggttcactacaaccaccacctcctgggttcaagcgattctccagcctcagcttcccgagtagctggcattacaggtgctcaccaccatgcctggctaattttttatttgtagtagtgacagggtttcatcatgttggccaggctggtctcaaactcctgacctcaagtgagctacccgcctcagcctcccaaagtgctgggattacaggtgtgagccactgtgcccagccaggcattttctttaaaatgttctgcatatatttcctatatgatcagacctttaagcaaaatatctgatcttcggaaatgcaaagggatttctgggtataggaaaagtcttgttttcttataattacaaaatatattttctacatcataaactgatagtaagtaagcatatcatgtccttgtaacaactaaacactggggcaaatatactgactgataagcccttatgaaagaatacacattcatgttataaaataaaatacatctaaaaccatggccaatattcagccaggaagtaccagtctgggcccataggctgtttctgcaaggcctgagttctggtcagtgtctgtgccttaccacatgttaaaaattttgattataatccctatgtatagtgctatagaaccactaatggataaacataaaaagatagctcaaaaatgtcagacataaaaagatattacaagctgggccaggcggccagcacctgtagccccagctactctagaggctaaggcaggaggactgcttgagcctaggagttcaaggctgcagtgagctatcatttggccactgcactctagcctgggcagcagagcaagacctagtctcttaaagaaaaaaaaaaggcattacaattaccaacaggtatctgtaagagaaacttgtgtctcttgctggtaccgaatagccttcctcaaagactgatgaagcactctcatgctaagaaatgcacatctgtaaatattatcaaatgcaggcacttagaatagtctagttaacaatttatagtaagctagtatatattaaagcaaaagcaaaatactgcctagatatgaatgttttagggggttgcttggctggtggccggcttgggtttcgcttgtacattcagcacataatcatgccggaaggatgaacgaacagtgcgattcatcagtggctgaagggggcggaagttgtccaccattcttttctctttctccccttcggaagtgaaaagcagggtccgaaattgctcaagctgatcatgatcaacctctactggttgcttcttaatgatccaggtgacagactcggagaggggtggggtagtcagagaccctgagtaggtccagtaatctgggcaggtaggcatcaggcaggaagggtcaaatgacccaaattccacaagggcgtccttatgcttaattgacggcaaagtatccactaatttctgtagctccttatgatgtttgcctagctttaaaaatactcctatcacagccaaaccattttcttccagtgctgcatcctcaaagttttcaaatctgactgcgttccaatgcactaagtgcagctctgctgggaagcatttgctgtccacggtgtgctcagaaccccaggcatcgatggccccccagtgaaaatggaactgcttcaatcggtagttgtgttccaggggtcctcccttgatcactgatttatctgtagaatcttcaaattccacgaggaaagagtacccattattccagacgtggaggcaggtggctgggtcataagagatggtcagtggttttaagccgggatcataaacactgtccctccaccgaatgttgatgggtgactggcgatcgcccccaggaaccaggtccacgctctcccagagtggatgcaaggctcggttccgggttttgtaagtacaagtatagaggctgcagggcctcgctggcatgaatctcggaatctggaactttctccacagcaatttgcctggagaggcttgaagaatgaccctcaggctgttcatcaccaccatctttagcttgaaatcttgatcagttcccagttaagttgcaggaacttaataatctgagcgtctctccagatcacgaacctagccgctcgctcgcctacggggatccgcagcctgcacgtccggccatcgaagctac

SEQ ID NO: 14034 - RNA, 7409 nt, Homo sapiens
  source 1..7409: mol_type = other RNA
gctgggattacaggcatgagccaccgcacccggccatagattttttagtgagttagaaatgaatgtaaatttccttttataggagttagacatttatttttaacaattaaccactgaattcattttcagaaataggcctgaattgcttgttaatttcattacaggaagtaactctaaaagccaattccacttccaaactataattaccatcatctgaatttaacagggaaagacatcttccaagacttcttttgggcggatgcttagttttagaatagccaactttaccctaacccatgtacaagacagttctccaggtggccttggactgacccagttctcccttcttccttgcttgtagttcttaagaataactgtagaatgcactgggaatgcaatatcctgatatggaggaactgcctgaaacaggttggccttgttgttgtccctcctagggaatgtaacatcttgatttagggaactgtttgagacagcgaggttgtgttcctctttcccctggaaggaggatgtactttaaagctttgcccaatgagttatgtggctcctatggtatataacccaaggcaggctgtggtgcaagtggggcacgtacaatcaagactccatcagccccgccctgggcagctttcttgagccctgggggactggctcacaatggagccagggcctcttttgtcccttgcttcctgtctgtaagtaataaatctgcttcatgtaatgtattgggtgtgagtgtgttctgtcacaatggaatcagacaggttggtaaccagtgtacactgaacctgcttggcaccatgtagccctgggaaaggagaaaggcggtcacagcttgccctatatggtgatgccagcacactgtgcactgtactgtgcaacagaaaaaggtgcactgaggaggatcggctgcttcttcccattgttgcttctttagtaaatcccctatgagtttttagtcgctttctaatctacaagttaaaggatatctcattaattttacagatatatacatatactgtaacaataggaaggaagtctttcaccaaccactaatactgtaaagaaagcattgtatcgatctagtattatttaatgaagacggacagcaattttaatacaatcttcttttccaagacctttgacagaccttaggcccattttccacctttatgtctaggaaagtataagtaaaacacttttgagggcataaaaaacacaagcttcttgttaaggtgtatcagtagccagggaaatctgctgtgcccctttgagggtcatctaactaaggcatggagaaagaaactgcctcaagtcagtttctatcacctctgcagggaagctggccatgcaaaccaggacatggttcaaagtgaaaaagagtgtggttaataatcatgccagaacaccaggtataagatgtaagggcaagtcaggcattctgtacattgcttctcccttcagtttggaaaactcactgcagtagggttttgacttatcgtttcacaagacagctaggaaggccaggcacagtggctcacacctgtaatcccagcactttgggaggccaagacgggtggatcacgaggtcagatcgagaccatcctggttaacacggtgaaaccctgtctctacttaaaatacaaaaaatagccgggtgtggtggcgggcgcctgtagtcccagctactcaggaggctgaggcaggagaatggcgtgaacccgggaggcggagcttgcagtgagccgagatcgcgccactgcactccagcccgggtgacagcgcgactctgtctcaaaaaaataaaaaaaataaaaaaaaataaaaaacaagacagctaggaggaaagcctgtatgctttggaaaatgcatatcttgtgtgtttacccttttaaaggtaactatactttgaaacaggtgaactgcagaaagttaacaaagacttctttttttaccatgtttacctttctaagaattctatgcatttcctagggcatacatgcaaaagccttcacatttccccctttttaaaagagatatttctcaaacttatacgtatacagttcagtagtgttaagtacaatcacacttgttttgcaacagatctctagaattcttgcaacacaagctctgtacccactaaatacaaattcaccctctccccttcccccaaccgttgcttggcaaccacctttctactttctattgtatgattttgactactttgcatacttcacatggaggaatcatatagcatttgttcttttgttggctggcttatttcacttggcataatgccttcaaggttcatccacattgtacatttgacaggatttccttctttttaaaggctgaataatattccattgactgtatataccacatttcctttatctattcatctgttgatggacatttgggatgcttccagaacctcttggctattgtgaataatgctgctatgaacatgggtgtacaaatatctctttgagatcccgctttggtggtaattcttatggtaattctgttttcagttatttgggaaacctgtgtactgttttccgtaatgactgcaccgttttacattaccaccaacagtgcacaagggtttcaacttctctgcatcctccccaatacttgttatttttttgttcttctgatagtggccatcatgatgggcgtgagacgatatctcattgtggttttgatttgcatttccctaataattggcaatgttgagcatattttcatgttcttattggccaattgtataacttctttggagaaatgtctgtgcaagtcctttgcccatttttaaaaattgagttatttggttttttgttgttgagttgtagaagttcctcatatattctggatttgggctccttataagatagacgatttgcaattattttctctcattctagagcttgcgttttcactttgttgattgcttcctttgacacacagacatttttaagtttgatgtagtcccgtttccttcctaacgatctttaagtgtacagttcagtagtgttaagtatattcatccaaccctatcttgcagaccagatgacaaacatattaatgaaagaaatactaccagtcattgacgcaacagagtctgaacataggcttagaggcattcagaaacattccaagatatttataagcaagagccacaggagcatgaattcctcagaatatgtagaattatctagattttagcctatctgacaagtttctctccctattaccataacaaaagtcttttaaaccactgtataaactgagatatttaagttaatcacctgccttgcaaagaaccttgactaatgagtaaataaagttcagacagttgtaaagggaagacgggatagctctttcactgtagaaaacattatcattatatactatgtaacagcgtgcaaataatacaaaataataatataaactataggctattagattactagtcctttgaaaaatatttctggaaggccgggcacggtggctcacgcctgtaatcccagcactttgggaggccaaggcgggtggatcacctgaggtcaggagttcaagaccagcctggccaacatagtgaaaccccatctctactaaaaatacaaaaattagctgggcgtggtggcatgtgcctgtagtcccagttactcaggaggctgaggcaggagaatcgcttaaacccgggaggtggaggttgcagtgagccaagatagtgccactgcactccagcctgggggacagagcgagactccatctcaaaaaaaaaaaaaaaaaagaaaagaaaaatatttctggaaatgtgcaatgaaagaattctaagttctaggcactttaagcattttttcttttcttttctttttttttttttattagacacagagtctcactctgttgcccaggctggagtgcagtggtgtgatcttggttcactacaaccaccacctcctgggttcaagcgattctccagcctcagcttcccgagtagctggcattacaggtgctcaccaccatgcctggctaattttttatttgtagtagtgacagggtttcatcatgttggccaggctggtctcaaactcctgacctcaagtgagctacccgcctcagcctcccaaagtgctgggattacaggtgtgagccactgtgcccagccaggcattttctttaaaatgttctgcatatatttcctatatgatcagacctttaagcaaaatatctgatcttcggaaatgcaaagggatttctgggtataggaaaagtcttgttttcttataattacaaaatatattttctacatcataaactgatagtaagtaagcatatcatgtccttgtaacaactaaacactggggcaaatatactgactgataagcccttatgaaagaatacacattcatgttataaaataaaatacatctaaaaccatggccaatattcagccaggaagtaccagtctgggcccataggctgtttctgcaaggcctgagttctggtcagtgtctgtgccttaccacatgttaaaaattttgattataatccctatgtatagtgctatagaaccactaatggataaacataaaaagatagctcaaaaatgtcagacataaaaagatattacaagctgggccaggcggccagcacctgtagccccagctactctagaggctaaggcaggaggactgcttgagcctaggagttcaaggctgcagtgagctatcatttggccactgcactctagcctgggcagcagagcaagacctagtctcttaaagaaaaaaaaaaggcattacaattaccaacaggtatctgtaagagaaacttgtgtctcttgctggtaccgaatagccttcctcaaagactgatgaagcactctcatgctaagaaatgcacatctgtaaatattatcaaatgcaggcacttagaatagtctagttaacaatttatagtaagctagtatatattaaagcaaaagcaaaatactgcctagatatgaatgttttagggggttgcttggctggtggccggcttgggtttcgcttgtacattcagcacataatcatgccggaaggatgaacgaacagtgcgattcatcagtggctgaagggggcggaagttgtccaccattcttttctctttctccccttcggaagtgaaaagcagggtccgaaattgctcaagctgatcatgatcaacctctactggttgcttcttaatgatccaggtgacagactcggagaggggtggggtagtcagagaccctgagtaggtccagtaatctgggcaggtaggcatcaggcaggaagggtcaaatgacccaaattccacaagggcgtccttatgcttaattgacggcaaagtatccactaatttctgtagctccttatgatgtttgcctagctttaaaaatactcctatcacagccaaaccattttcttccagtgctgcatcctcaaagttttcaaatctgactgcgttccaatgcactaagtgcagctctgctgggaagcatttgctgtccacggtgtgctcagaaccccaggcatcgatggccccccagtgaaaatggaactgcttcaatcggtagttgtgttccaggggtcctcccttgatcacttctcttataatcctatcaaggtaggtaggtcatgttgtcctctctttcattccagagtttagtaatttgagtcttcttttatttttttcttggtctcccccaattaaaagtttgtgaactttgttgatcttcccaaagaaccaacttttgatttcattgatttctgctcgttctttattatgcccttctctctacttgcttttgggtttagtttgttcttctttttctagtttcttaaggcggaaagctgagatactgacttgagaaagttcttctctattgtaggcattttcatctatacatttccctctaagcactgctttagctgcatcccaaaaggactggtatgatgtttttgtcacataccttccccagctccttttccttgcactttattccaatcctcacaaagcacactgtggcagcatttcttagggttttgtctttgaaatttatagacatcgatatttattaggtttttacttttctagaattgtttcttgcctttgtttctaaaatgtcttgctttctttcactttttattttttatgttcattcactctttttttcctctttgcatgctattgattgttttgcaacaacatggagaaatagcagcaaagaataaacaggaaataagaggcagtcactgatttatctgtagaatcttcaaattccacgaggaaagagtacccattattccagacgtggaggcaggtggctgggtcataagagatggtcagtggttttaagccgggatcataaacactgtccctccaccgaatgttgatgggtgactggcgatcgcccccaggaaccaggtccacgctctcccagagtggatgcaaggctcggttccgggttttgtaagtacaagtatagaggctgcagggcctcgctggcatgaatctcggaatctggaactttctccacagcaatttgcctggagaggcttgaagaatgaccctcaggctgttcatcaccaccatctttagcttgaaatcttgatcagttcccagttaagttgcaggaacttaataatcagattatgtggagtagaaatagtcccattacagtaaggaagaagacaagtgtccatgttatcccaccattatgtcactctgttgtgatagtgccactttaaaaatactcctatcacagccaaaccattttcttccagtgctgcatcctcaaagttttcaaatttgactgcgttccaatgcactaagtgcagctgatttatctgtagaatcttcaaattccacgaggaaagagtacccattattccagacgtggaggcaggtggctgggtcataagagatggtcagtggttttaagccgggatcataaacactgtccctccaccgaatgttgatgggtgactggcgatcgcccccaggaaccaggtccacgctctcccagagtggatgcactgagccagaacctcctcgttcgctcccggtacccgaggatcccgcacgcggccatcttggccacgccccctcacgtttagccacgtccctacgcagcaaacgtcatttcgtcattccaggttacgcccctatcagtccccattctgtccccgacccaggctgaaatctcgccctggccacgcttccccagcgccggagtccacacctgctctgcgctctggctacacatctcctgtcgctgccacgcgcctgcacgctaacttgccgacgcctctgccctccgcctgctccaccatctttgttacgcccctcagagcaac

SEQ ID NO: 14035 - RNA, 4387 nt, Homo sapiens
  source 1..4387: mol_type = other RNA
gctgggattacaggcatgagccaccgcacccggccattttcactcttaaatactatcaggcacacagtatgcaaaagacactgtagtaggcacacagcatcggtgcttagttattgttaacaacccaataattataataatggtgatgtcaacaaatacgtgttcactatgctgctttagagtttgaaaaaaagttataaaattattttcttagaatttgagtcagatagataaggaaagtcttgttttaaaaaataatataagtagagcttatttgagccaagctttaggattgcaacccaggaacatagattcaagttgccctggatacacactctataagcagcagttacaggtggatttttactccagactgggcaacagagggggatcctatctctgataagagaagtcttttaaatcttaattttaattggaagataatggcgattgtaactggcccaagtaaataacagatagttacaggaatgttattcaggtcttttaacaccaaagatctggtgtcccctgctgcagttaccaatgattcttatcttttcaaaaataatttttgattcctaagtagtaaaggtgaaagatctcttgtatgaacgtctgtcgtttatagttatcaagtaacactgagaaaaaacaaaatctttttttttttttgagagagagagagaaaaagtctcattctgtctcccaggctagggtgcagtgacacaattatatctcactgcagcctcatacccctggacttaagcaatcctcctatcagagcttctcgagtagctgggactacaggtgtacgccacacatctggctacttttttttctttttggtagagacagagtcacccaggctggtctcaaactcctggtctcaagggatcctcctgcctcagcctcctgaagaggtgggattacaggcgtgaaccaccatgctagctaaaaccaagatcttgatctttaacactgacctaaattaaggttattttttttcccacattagaaaaagaaagaaccttacaaatgtcacatagtaggaaaaaacctaagaaacgagatgtactcaatccaagacacaaatagtttgccaagaagagaaaggtaaagaaaaactaggacatgcattattttcccccacaaaattaagacttcagaacattcttttgatataaaagaaaaacattagaattatgtgactctctgcaaagggctaagaaaactaagcactaatcaaagacaatcttgaattttcctgtcaaccaataaaaacgataccctcggccgggcgcggtggctcacgcctgtaatcccagcactttgggaggccgaggcgggtggatcatgaggtcaggagatcgagaccatcctggctaacaaggtgaaaccccgtctctactaaaaatacaaaaaaattagccgggcgcggtggcgggcgcctgtagtcccagctactagggaggctgaggcaggagaatggcgtgaacccgggaagcggagcttgcagtgagccgagattgcgccactgcagtccgcagtccggcctgggcgacagagcgagactccgtctcaaaaaaaaaaaaaaaaaaaaacgataccctcacctgaacaagggagtcttccactttacaaaatcacgaatcttcctgtaccaaaagaggttcgcttctataacagccgatctagctgatgagcctgtctgattagttgggttgcgggaagatcagattactcttcccgcttaggcggaaagaaactcacctgaagttgcctgggttctcctttcgtttcaagtaaatcctgagttatcagaagaggctcgcttttctcatagctctcctggttgataagcgtgtcggcatagttgggctgggggaaaatcagatgactcttacgcgagtctgcagtgagtgagacctcgtgggaataggtctgcaggaaagcccgaaccccttccacgcccacaaagtgcgagccgggcatgctcgctaagccacctcccgaagcctgcagcaggcgtgacttgtgccagcgctgcagtctgagcgccagcagcacgatgacgaaggccaggaagacgcaggagaccgcggccaccgccaccaccaggtacagagtgaggtccgaatcgttgggtttggcggagggctcgaggctgcccaggtcggccaggatgtcggggatcctgtcggccacggccacggtgagcgtgacagtggcggagagagggggctggccgtggtcctggacggccaccactaggctctgcttgagcgcgtctctgtccagcagggcgcgcgccgtgcgcacctcgcccgtgtgcaggcccactgagaaaagtcctggctcgctggccttgagcaggcggtaggacagccaggcgttctggcccgagtctctgtccaccgccaccaccttggtcaccaggtagccgggctctgcggagcggggcgccagctccacgccagtggaaccgtctgtggggagggcggggtacaggatctcgggcgcattgtcattctggtccagcacaaacaggctcagtgacacgttgctgctaagaggcgggtccccgctgtcgctggctgtcacccacagctgtaggtctctcaactgctcatagtcgaaggagcgcagggcgtacagaatcccagtgtcggagttgatggacacgtaggaggacaggggcgccccctggagggtgtcttctgccagtgagtaggagacttgggcgttctggtccacgtcagggtccagtgcattcacagagaagatggaggcacccctggggttgttttcaaggacatagactgagtaggatgaatgggggaaggtgggcgggttgtcgttggtgtctgccacatttagagagatgattgtttctgtagacagaggtggtgttcctttgtccgtggctgtcacagtgatgttgtacaagaatacctcttcccggtctagagctgcatttgtcactaatcgataataattgccaactgatttttccaattcaaatgggagacttctcgggatggaacaggttaccaggccattcaggccagagtctcgatcgaacacttgaaaaagggcgattactgttcctggaggtgcactttcagcaattgttctgcttccagatgtaacaaccacttctggtacattatcattgacatccaagatagttattaagactttcgctctgtctcgaagacctggcccatcccgggcttcaacacccagctcataaaaactcgagtcctcatagtctagatttgcagaagttgaaatttctccagtcaaaacattcaaacagaaaatttgtgagatcttttctgtaatcttcacaaaggaataagttacttccccgtggactccttcatcctggtcggtggcagtcactgccaacactggtgtgcctactggcaggttttcaggaacacttacacggtagacaggctgagtaaacattggagtgttgtcattcacatctagaactgttaccagaatttgggcgacgcttgagcggacagggtcgccgccatccatggcagtaaggaccaggcggtaaacggcttctccttcccggtccagtgtgccctccagcaccagctccgggtacttgggcccatgggcttcgctttgcacgtccactgagaagtgactattaccactgagcttaaatccctgaagggagttcattcccacatcagggtcatagacctccattagtggaaaacgagaggatggagctgcgttttcgagaattttcacttccaattcttcctttaagaatcggggtgtattgtcattaatgtccactatttccacttccacgggataaagattcagtttatcctcgacaaggatgttaaaactcaccagacaccgcgggctctgagcacagagctcctcgcggtctatcctacccgcggtgaccaagctgccgtttcgcggattcagagagaaaagctgcatcctacctctggagacgatgcggactccgtgctccgccaactcctggggctccagtcccagatccttgacgatgttgcctacgaaggagcctttctccagctcctcgggaatagagtagcggatctgcgctgccgcggccccccacagcgtccccaggagcgtgaggagcaggacctgctcgctgcgctgcggatgcctctgcggaggcgccattactggcttattaggaacttctctgggattaagaagaggaagaacagatctgcatcacttttgctcttctcagaaatagcggtgaaggtccttcaacaagcagagaccggatgcgaagcgtttcaggtcagaatttctgcacagctttcctgctttcccgtctaatttgctttgttgttggaggatgtaactt

SEQ ID NO: 14036 - RNA, 1303 nt, Homo sapiens
  source 1..1303: mol_type = other RNA
gctgggattacaggcatgagccaccgcacccggcccagttcaggaattcttcacgcataactagaccttcttgctatgcccttaggttcaacacttttaggtcttcctttgcacacatggaggactgtgatttcttagatcttcaaatttactcctgaagagaggcagccaagaggttttccagctcgtgccaggagcgattggcaggttcgagcagcacagtcattccgcacacagatgtccctgcgttcactcttctgatatgaattctgtcagctccgaatccgagagagacaagcagacagctacacagacagagtcacagacagacacagacacagatagagcaattgtctggaagacgcagaactctacagatatttttcttccctgcccagacatttcagcggccccaagggccccacaacatcatcacggagcttcaaagttaagtggtggcagagagaaactctaaagtccgcgagatctgtcccctcacgcaggacccttttgtagttctagaaatccagtatccctgagagttctagaacaccaccaaggtgcaagttccagcattctagaacctctgaaattcaaaattccagaactcccatgaattgcaaatcgtgctgagtgcccagttcttatattgccctcttcgtgggtgcgcgggaagtggatgctgtccggtgccccgagcggttcgcactgcatgcctggtcctcaccggctgcctccagaaccttggccaccagccaaaagtgcagcctgccctttgatttaggaacacagaaaggtcaagtctccctggctactgtccctttctgacgttgccttccagagcggaccccattcctgctcctgtcccaccctggccctccacgcctgacctggctgtcctgcctctgcccctgccagcggctgtgggagtgagctggttggtcactgggcatctgtgagctggctgggcatgaacagccctggggtttggttctccctggtcatccctacttagtggacgaagaaaaagggggcaaagaaactggtcacgacagaggagggggcacagaggggtttgggctgtggtttgtggggttgtgttttttaatctttcctactttctttttttaaaagaaaaagcccccatcctgtgtcatcatttttatgggatctgcaattctggcaaaaatctgtctttaatttagctgtccatataaaaatcctcactgtataataatgaacagatgccatggaatttaagctggagcctcggctcctccccgccttccccccgcgcctggca

SEQ ID NO: 14037 - RNA, 2694 nt, Homo sapiens
  source 1..2694: mol_type = other RNA
gctgggattacaggcatgagccaccgcacccggccctgttttcttcaaagcatttctcaaatgtgtataatgagaatttggggactggtaagggctttggagatcattgaatccagcacgcccatcttgcaattcaagcctgcaaactgaagcctagtaatgtaacagatttacctaaggtcccacaggtagaaagtgaataaatattctggtctactgttatctaaaccagtagcatttttactatcctttctgtgaatcatattcagtataacagtttactcatctgacaccatcctgtgcttttatcacaaaaatccaggttttgtctttatttgaaactgtaacctgtaataataattcagatattaaatatactataatgcatacagttgtttcattcgtgttttataaaggtagtttttgtgtctatttttgtaacacctactgatccttactaaaacatctgaatatctaagacctcctgtaacacagttgatcagtttgtttcaatcatcccagtagctaatgtgcattactttactgttacccaggctgtgataattagttataaggattatgtttgctgcaatggactgactattctccaggcccatatctctactaaatgggctaacatagaacaaagacaaggcagtggctaaattttcactttaatcacaaatcatcttgactaaaagttcacatagctcaaatctgagatagctgttagactttcattttttcctgtagtgatctagtctcaaaattttgacacaaagaaattaccagcagattgtgagacattcattgtagactttgcctcaaagaaagttacctagattgtatctcttatttatctatctgtttcgctgcaggtataagattgttttagttactgattctcatacaatgcaattcatcacttttactccattctgtaggggatcaaaacatttataatcttggctttgctactgaaatatttttatagttactaaaattctacaagtgctcttattataacatagcatggttatatatttaaataacagaggattggttatttatgcatttgttcaggtatattttgaaactaaaatatggaaataaaaaagggttctatataataaattttcacagtttgactttccataaggcttatgaaataatatacaaatagctaccattctgctgaaatgtcacagtaaatacattaatggcacagaagtgaaatgtccccaaatgggaagccatcttcatgacctcctaaatctcttttccaactaaaacttttttttaattgaaaaagagttccatttctaaaagaatataaaaatagaaaatgagttaaggaaacttttacatatataattttgaaggaaaagctataaacattagatgaaatattatatatatctttaagaatgtgctttgtctcaccacaccaaacatcccatgaaaacaaaattaaatgaatatattatatatgaactgttgaaagtataactaaatgttacaattttaattaagatagaatattaaaacatgtagtaagtactaacacatttttgtcaagttcagctcagctaaaacctataaggctaatttgcaaatttatcattttgattaaaaaataaaagaatgtttaatcaagcaaggcacatttcttttaggcaagtctgtctttaataccattcatttgggcacagtgtagacttcacttatttatatgtaaatgggctaatctatgtatgagagcctttggtacaaaacacaccttcacaaataaagttgcacataacccagaacatggaatataacacgactatatctcatgattaaacacagtccactacttaattgaaaaaaaaaacacaaaaaacagtaatagttggcttgctagaaacaaattttaggctttctttctgcagcactgattatagtttttggatgattcgatttcatcaaaatgtcaaaaggttgcaatgataccttaatatttttagcattcttcatctcttgatgaaatgtcttttatatgcacgcattatgaagcgaatcctccaacttcagagttgttccctttatataaagcatttgttagagacatattatttaatgtcaactgaaataaaaatatgtgctggcagatggatcactgcccatcagtgatataactgctactgcattcttgatccaggcaatttaaaatggagcatcctactggtcagtgcagctctacagttctttatatggggggctcttcagggatctctatctcacagtgtttccataagtcttcagattatggggcacgtgtgcttctttgcatttcttagtgggaagggttatcacttctattcacagctgagaggtgggaaggacttggaactgattctgtctgtcttctggcaacccttggcatatggctgaaacttgcaggtgttctcccaagatctggttacttcctgtccctccttttaattgattgtctgcaattcactcagttttaaacgtgcatcctttatttatttgaagtttatttagcttgtcaagtgctgtgatgatgacagagctgttgtgggatctgtatttttttttttaaagagaaagcctgaaggtcccttgtagtaaggtttcaggcacactgatcgaatctctcatttgcttatgtacagaacacttttacat

SEQ ID NO: 14038 - RNA, 2615 nt, Homo sapiens
  source 1..2615: mol_type = other RNA
gctgggattacaggcatgagccaccgcacccggccctgttttcttcaaagcatttctcaaatgtgtataatgagaatttggggactggtaagggctttggagatcattgaatccagcacgcccatcttgcaattcaagcctgcaaactgaagcctagtaatgtaacagatttacctaaggtcccacaggtagaaagtgaataaatattctggtctactgttatctaaaccagtagcatttttactatcctttctgtgaatcatattcagtataacagtttactcatctgacaccatcctgtgcttttatcacaaaaatccaggttttgtctttatttgaaactgtaacctgtaataataattcagatattaaatatactataatgcatacagttgtttcattcgtgttttataaaggtagtttttgtgtctatttttgtaacacctactgatccttactaaaacatctgaatatctaagacctcctgtaacacagttgatcagtttgtttcaatcatcccagtagctaatgtgcattactttactgttacccaggctgtgataattagttataaggattatgtttgctgcaatggactgactattctccaggcccatatctctactaaatgggctaacatagaacaaagacaaggcagtggctaaattttcactttaatcacaaatcatcttgactaaaagttcacatagctcaaatctgagatagctgttagactttcattttttcctgtagtgatctagtctcaaaattttgacacaaagaaattaccagcagattgtgagacattcattgtagactttgcctcaaagaaagttacctagattgtatctcttatttatctatctgtttcgctgcaggtataagattgttttagttactgattctcatacaatgcaattcatcacttttactccattctgtaggggatcaaaacatttataatcttggctttgctactgaaatatttttatagttactaaaattctacaagtgctcttattataacatagcatggttatatatttaaataacagaggattggttatttatgcatttgttcaggtatattttgaaactaaaatatggaaataaaaaagggttctatataataaattttcacagtttgactttccataaggcttatgaaataatatacaaatagctaccattctgctgaaatgtcacagtaaatacattaatggcacagaagtgaaatgtccccaaatgggaagccatcttcatgacctcctaaatctcttttccaactaaaacttttttttaattgaaaaagagttccatttctaaaagaatataaaaatagaaaatgagttaaggaaacttttacatatataattttgaaggaaaagctataaacattagatgaaatattatatatatctttaagaatgtgctttgtctcaccacaccaaacatcccatgaaaacaaaattaaatgaatatattatatatgaactgttgaaagtataactaaatgttacaattttaattaagatagaatattaaaacatgtagtaagtactaacacatttttgtcaagttcagctcagctaaaacctataaggctaatttgcaaatttatcattttgattaaaaaataaaagaatgtttaatcaagcaaggcacatttcttttaggcaagtctgtctttaataccattcatttgggcacagtgtagacttcacttatttatatgtaaatgggctaatctatgtatgagagcctttggtacaaaacacaccttcacaaataaagttgcacataacccagaacatggaatataacacgactatatctcatgattaaacacagtccactacttaattgaaaaaaaaaacacaaaaaacagtaatagttggcttgctagaaacaaattttaggctttctttctgcagcactgattatagtttttggatgattcgatttcatcaaaatgtcaaaaggttgcaatgataccttaatatttttagcattcttcatctcttgatgaaatgtcttttatatgcacgcattatgaagcgaatcctccaacttcagagttgttccctttatataaagcatttgttagagacatattatttaatgtcaactgaaataaaaatatgtgctggcagatggatcactgcccatcagtgatataactgctactgcattcttgatccaggcaatttaaaatggagcatcctactggtcagtgcagctctacagttctttatatggggggctcttcagggatctctatctcacagtgtttccataagtcttcagattatggggcacgtgtgcttctttgcatttcttagtgggaagggttatcacttctattcacagctgagaggtgggaaggacttggaactgtcagagtcgagttactccttgcttttcggagctcctcggctgaagaggagaggtgctggcaacttcccacgtgcatgtactgggattgctcttccccttctgtctcccggtggtagaagtaattgaagttggaaacaatcacgggaactggcaatgcgatggtcaagacaccggcgatggcacagagagatcccacaatcttgccccctatggtcact

SEQ ID NO: 14039 - RNA, 1859 nt, Homo sapiens
  source 1..1859: mol_type = other RNA
gctgggattacaggcatgagccaccgcacccggccgtcttttagttatttttttaaaaaatatttacatctgggctcctaaacgtgtttatgttgtaatgtttgatttgtcagtgttactgattatccatggacttctcttgggggctgtgaggactgagcgtgcctacacctgtgtaccccaacttcctctccccccagctccctgcccatacttagaacctagtttgggtgacatcagctgtcagggttgtgactgggtgcatactggccattgttgaacctggtgtggtggtgcaggggatggttttctttcttacagcatcttttttcgcccgagttagtaaatgctcaaaactcaggccccacgtgcagcccctgccccctgctccccatgccagccgcctggctgtcatccggggaccctcctgccagcttccatcctcccccgtctccccgggcctcagctacgtgaacctcagcacgctgtctgtggcgagaagccggagtgctcatggagctgccgcagcagcctggtgacagggcagggcctcgctgtcctgaccctccatccttggctgttggtttttatcctcctgttggtggccttgtgatcacagctgctgccacagctgcagacacgacgcttgcagaccagggacagagaagggctcagccagggagttcctttctcacctgtgtctcttatccaaaaaccaatgtttccagaagtccctgcagacttcacggctgtgaagggggctggggctgtgaggcttaccagggggagcgccctgccacagccccgatcccggtgagtcctcagggcccacagagccttctggagcagcctgtctgcgggaagccccctccgctggatctggtgaaacccaggggcgctttcttcattcccacccttccatctccttgtgttttctgtgtggcttttctgaagatcacaccagtgcttactgttttccagccgcacaatggttgtcttttcactgcagcgttcagcgcacccgtgttgagggggtttctgatgtggtgggtgtaagtccccgtggccgggtggggcgcttcgtccaccactgctccctctcgtgtgcgcttcctcgcacttccctgatcggctgatcagtctgcagcatttgtcgtctttcgcacggaagagctgctgtgaggtggaggcgggactcgagcgtgctcaggaacgggacgggagccgccctcattctccagcgtcctccgtgccaggcttcgtgcaaatctgtgactcttcctgtcctgggagctccatgcaagtgcagccggacagcacgtggtctcgtgacaggcttcctgcattggcattgtgttttcgaggttcatccgtgctggagcaggtgtcagaactgccttcccttttaagattcgatcatcccacaacacgtgtcttttcaagctggctttttgaatttcaccatggagcccagattgcaggagcgggggccagtggagtccgtcctgtagccaagaagcaggcaagagaggctgggacccatccctgcagctggggcagcagtgctgtgagctgtcagtgcttagtttatagacatcatcctgggagggagaagtgatgaagtagaaaagacgcagaagaaaagatgggacgtttgggagtaaacccctgaccaaaggcaagtaaggaaattccaccctgtgcagggggagcggctgccatgtccagcccaccctagacatggctgtggcctggcagagcagctcctgggtgggccttcccccacttctcttttttttttttaagacagtctcgctctgtcgcccaggctggagtacagtggtgcaatctcagctcac

SEQ ID NO: 14040 - RNA, 1971 nt, Homo sapiens
  source 1..1971: mol_type = other RNA
gctgggattacaggcatgagccaccgcacccggccgtcttttagttatttttttaaaaaatatttacatctgggctcctaaacgtgtttatgttgtaatgtttgatttgtcagtgttactgattatccatggacttctcttgggggctgtgaggactgagcgtgcctacacctgtgtaccccaacttcctctccccccagctccctgcccatacttagaacctagtttgggtgacatcagctgtcagggttgtgactgggtgcatactggccattgttgaacctggtgtggtggtgcaggggatggttttctttcttacagcatcttttttcgcccgagttagtaaatgctcaaaactcaggccccacgtgcagcccctgccccctgctccccatgccagccgcctggctgtcatccggggaccctcctgccagcttccatcctcccccgtctccccgggcctcagctacgtgaacctcagcacgctgtctgtggcgagaagccggagtgctcatggagctgccgcagcagcctggtgacagggcagggcctcgctgtcctgaccctccatccttggctgttggtttttatcctcctgttggtggccttgtgatcacagctgctgccacagctgcagacacgacgcttgcagaccagggacagagaagggctcagccagggagttcctttctcacctgtgtctcttatccaaaaaccaatgtttccagaagtccctgcagacttcacggctgtgaagggggctggggctgtgaggcttaccagggggagcgccctgccacagccccgatcccggtgagtcctcagggcccacagagccttctggagcagcctgtctgcgggaagccccctccgctggatctggtgaaacccaggggcgctttcttcattcccacccttccatctccttgtgttttctgtgtggcttttctgaagatcacaccagtgcttactgttttccagccgcacaatggttgtcttttcactgcagcgttcagcgcacccgtgttgagggggtttctgatgtggtgggtgtaagtccccgtggccgggtggggcgcttcgtccaccactgctccctctcgtgtgcgcttcctcgcacttccctgatcggctgatcagtctgcagcatttgtcgtctttcgcacggaagagctgctgtgaggtggaggcgggactcgagcgtgctcaggaacgggacgggagccgccctcattctccagcgtcctccgtgccaggcttcgtgcaaatctgtgactcttcctgtcctgggagctccatgcaagtgcagccggacagcacgtggtctcgtgacaggcttcctgcattggcattgtgttttcgaggttcatccgtgctggagcaggtgtcagaactgccttcccttttaagattcgatcatcccacaacacgtgtcttttcaagctggctttttgaatttcaccatggagcccagattgcaggagctttgaagagaggaaacgcttgctcagtgggggccttgagggtggccatgtgtcggggctcaggggccatttccagaaggcgttgccctgatgctgccacttgctccctgcccgggggccagtggagtccgtcctgtagccaagaagcaggcaagagaggctgggacccatccctgcagctggggcagcagtgctgtgagctgtcagtgcttagtttatagacatcatcctgggagggagaagtgatgaagtagaaaagacgcagaagaaaagatgggacgtttgggagtaaacccctgaccaaaggcaagtaaggaaattccaccctgtgcagggggagcggctgccatgtccagcccaccctagacatggctgtggcctggcagagcagctcctgggtgggccttcccccacttctcttttttttttttaagacagtctcgctctgtcgcccaggctggagtacagtggtgcaatctcagctcac

SEQ ID NO: 14041 - RNA, 3365 nt, Homo sapiens
  source 1..3365: mol_type = other RNA
gctgggattacaggcatgagccaccgcacccggcctaaaaattcttgagaaattggaatgctaagttacatactaaatatcatcccaacagtaaggccgtagaacatatttgaaatcaagaaaaatgtgatttttcggttttaacacgttaagagcctctgtaacttttaaggaagctatttttttttctagagtatgcacatggtgatgatgtgttgggttgataaagcactggctcagtcctacaggcactaaacttcaatggatactttgttaactatagttacactaactttaaagaaagttcttgatacctgttctttattcttaggaactgaagaggagggaactccggtgtttgcataatcatcgccttcccatgttaagaggactcaccctagtaggcttaatgggttttgtatttggttggcttgttttcccaagagacactaaagttgttcttgcattaattccccttaaaattgccaagagataagaggtgggaagacaaaaagggcgcctgattctattcagtagatgagaaaatagatttacagaaggtaactgtgaaattggaggagtaatgtcagggaggccttgtcaggacaggcaatgtcaaggaagcctatcccttctttgtcagactccagaaaggattgagttcatctgttcttcacagatccactttcctaggcagatgccagtgccttccaggtttgtatgaaagcaaaaaactgctgacgatgggcagagggcctgtcccaaaccactaggaagcaggagagggcaggaatctcagtgaatcccagatgtatccacctgtgctgaaggctaacccccaacctgtttggtgatgtgtgagcagccagttggtttcatgggtcagaagagtgtggtaatggtacctggaatcctgcaaaatgcatggaaacaaggaagagcagatccttattccaacatgaacagcaggacttataaggaaagcaggcttttccccatgacctcacagctctgcctccacctttcatctcttcacagtgagctttctttcagagtgatcttaccacccaaccaggcacagtctaatttgatcataacaaggaggaggccgggcacagtggctcatgcctataatcccagcactttgggaggctgaggtgggtggatcacttaagcccaggagtttcagacgtacctgggcaacatggagaaaccctgtctctacaaaaattagctgggcacatggtggtctatgcttacagtcccagctactcagttggctcaggcaggaggattgcttgagcccgggaggcagagtttgcagtgagctgagattgtgccactgtaatacagcctgggaaacagagcaagatcctgtctcaaacaaaacaaaacaaaaaatcaccaaataaacgataaggaagtcaccctgtccaaggaatgccgtttcatatggtgccaccccttctcctagaccaaagttcccattttagaaataactccatgctaggcaaggttgtaacggaaaagaaaggctctacctccagcctcccagatcaccccatctctactggctctccagaacccagtggggctcatagctattcctaagccaggccacaattcctgccagcccatgactagatccaaagcccgtgcaacagcgagaggagcaggggccgggcggggggggggggggcgcggtgtgtgcctttaaagatccggattatggtctttagcctgggttcaactgtagcacaaccaaccaccacggacgaccaatgaccgctatgagacagttcttcctttcacacagcagcatcatttatctggtagtagcaagacagccgtatgactttttgttgttgttaaagaaaaataagttgtcaagatttgcctaccaataactttcctatgtcttggctttcatgtccagtgggctagtttccaactgtttgagactcagggtaatcccagaaacctgtgaagcatcggcacaaaggttgtagcgcagatgccaacagatgtgtaggtaacaaacttgtaaggcacttcaatctccagtctccgcctggcctccttgttcctggtgaccaccttgaaccatgagtataatacttgcagtgagagattttgtacaagctgacgaaccaagaggatcaacacaattcccactgcaaatttggtcagacccaaaactaacatgtaggtggtgagtggtgggatgttctgaataacagggagagattcagcgggcttggatacaagctggaagaaatggttgatccagaatcctatggtcactccagccccggcagccagaatggtggtggtgtccgcccgggttgggctgtagtaatcagaaacagggtaattgtaacacaggaagaatggcacaactatgacacacacggggaagagggggctggccgagtccaggcagtcgatgaaggtccaggcagggtaggtgaggacgatgaggagtgcggtgatcaggacgccacccagcacatccaggaccgtatgcatcccagtgtagagcctgctgagacacaccaaggtggaaaacaccacggccatcaccagtcccaacacaaatggatactggtatctgtccatagtagagataaggagggtgaaggcaatggcagtggccgccatggcgtgggtggatggcattccatattcagcgatcagtctcttttccagttttacaactggaggggaggagggacggggccacttcaagacatccttggccacttggccaatatacatcaccaaaacccatatgatgatcaatcttctggataaataagggtcaatattccagtgagtgaatggaagaaacgtgatgtagaacacttcttggcccaaagcagctgaaaattggaataggtaatagtagaaataattcttcacgacgtacttctgtacataagccggacactacccactttcttgtggcttgttagcagaactcaaactcaggccaaacctcaggcaatagtgcaagtcagtctggcaattcaacttccttctttcccaacctcatttgcaattaggggtggccatgacactcagtcctccggcgccgcggctctgcgcagcccgttggccggagcctcgccgcccttgccgttggctgcggggagatgctcgaccccggggacccgcgccgcgcgctccgtggggtccgcgccgttctcccgggggccttcatccggagcggggaagagcccgcagcggcgctggaagcgggcgacgagctgggaatcctgcaggctccgcagcagctcggccatggtgtgcccggggccgcgctccgccgccgctgccacgccgggccggtgccctccgctggc

SEQ ID NO: 14042 - RNA, 3160 nt, Homo sapiens
  source 1..3160: mol_type = other RNA
gctgggattacaggcatgagccaccgcacccggcctaaaaattcttgagaaattggaatgctaagttacatactaaatatcatcccaacagtaaggccgtagaacatatttgaaatcaagaaaaatgtgatttttcggttttaacacgttaagagcctctgtaacttttaaggaagctatttttttttctagagtatgcacatggtgatgatgtgttgggttgataaagcactggctcagtcctacaggcactaaacttcaatggatactttgttaactatagttacactaactttaaagaaagttcttgatacctgttctttattcttaggaactgaagaggagggaactccggtgtttgcataatcatcgccttcccatgttaagaggactcaccctagtaggcttaatgggttttgtatttggttggcttgttttcccaagagacactaaagttgttcttgcattaattccccttaaaattgccaagagataagaggtgggaagacaaaaagggcgcctgattctattcagtagatgagaaaatagatttacagaaggtaactgtgaaattggaggagtaatgtcagggaggccttgtcaggacaggcaatgtcaaggaagcctatcccttctttgtcagactccagaaaggattgagttcatctgttcttcacagatccactttcctaggcagatgccagtgccttccaggtttgtatgaaagcaaaaaactgctgacgatgggcagagggcctgtcccaaaccactaggaagcaggagagggcaggaatctcagtgaatcccagatgtatccacctgtgctgaaggctaacccccaacctgtttggtgatgtgtgagcagccagttggtttcatgggtcagaagagtgtggtaatggtacctggaatcctgcaaaatgcatggaaacaaggaagagcagatccttattccaacatgaacagcaggacttataaggaaagcaggcttttccccatgacctcacagctctgcctccacctttcatctcttcacagtgagctttctttcagagtgatcttaccacccaaccaggcacagtctaatttgatcataacaaggaggaggccgggcacagtggctcatgcctataatcccagcactttgggaggctgaggtgggtggatcacttaagcccaggagtttcagacgtacctgggcaacatggagaaaccctgtctctacaaaaattagctgggcacatggtggtctatgcttacagtcccagctactcagttggctcaggcaggaggattgcttgagcccgggaggcagagtttgcagtgagctgagattgtgccactgtaatacagcctgggaaacagagcaagatcctgtctcaaacaaaacaaaacaaaaaatcaccaaataaacgataaggaagtcaccctgtccaaggaatgccgtttcatatggtgccaccccttctcctagaccaaagttcccattttagaaataactccatgctaggcaaggttgtaacggaaaagaaaggctctacctccagcctcccagatcaccccatctctactggctctccagaacccagtggggctcatagctattcctaagccaggccacaattcctgccagcccatgactagatccaaagcccgtgcaacagcgagaggagcaggggccgggcggggggggggggggcgcggtgtgtgcctttaaagatccggattatggtctttagcctgggttcaactgtagcacaaccaaccaccacggacgaccaatgaccgctatgagacagttcttcctttcacacagcagcatcatttatctggtagtagcaagacagccgtatgactttttgttgttgttaaagaaaaataagttgtcaagatttgcctaccaataactttcctatgtcttggctttcatgtccagtgggctagtttccaactgtttgagactcagggtaatcccagaaacctgtgaagcatcggcacaaaggttgtagcgcagatgccaacagatgtgtaggtaacaaacttgtaaggcacttcaatctccagtctccgcctggcctccttgttcctggtgaccaccttgaaccatgagtataatacttgcagtgagagattttgtacaagctgacgaaccaagaggatcaacacaattcccactgcaaatttggtcagacccaaaactaacatgtaggtggtgagtggtgggatgttctgaataacagggagagattcagcgggcttggatacaagctggaagaaatggttgatccagaatcctatggtcactccagccccggcagccagaatggtggtggtgtccgcccgggttgggctgtagtaatcagaaacagggtaattgtaacacaggaagaatggcacaactatgacacacacggggaagagggggctggccgagtccaggcagtcgatgaaggtccaggcagggtaggtgaggacgatgaggagtgcggtgatcaggacgccacccagcacatccaggaccgtatgcatcccagtgtagagcctgctgagacacaccaaggtggaaaacaccacggccatcaccagtcccaacacaaatggatactggtatctgtccatagtagagataaggagggtgaaggcaatggcagtggccgccatggcgtgggtggatggcattccatattcagcgatcagtctcttttccagttttacaactggaggggaggagggacggggccacttcaagacatccttggccacttggccaatatacatcaccaaaacccatatgatgatcaatcttctggataaataagggtcaatattccagtgagtgaatggaagaaacgtgatgtagaacacttcttggcccaaagcagctgaaaattggaataggtaatagtagaaataattcttcacgacgtacttctgtacataagccggacactacccactttcttgtggcttgttagcagaactcaaactcaggccaaacctcaggcaatagtgcaagtcagtctggcaattcaacttccttctttcccaacctcatttgcaattaggggtggccatgacactcagtcctgtcagtgagaagtagggaggtgggtgggtcagaggcaagatcttctggatatgcttttgttttctttataaa

SEQ ID NO: 14043 - RNA, 3222 nt, Homo sapiens
  source 1..3222: mol_type = other RNA
gctgggattacaggcatgagccaccgcacccggcctaaaaattcttgagaaattggaatgctaagttacatactaaatatcatcccaacagtaaggccgtagaacatatttgaaatcaagaaaaatgtgatttttcggttttaacacgttaagagcctctgtaacttttaaggaagctatttttttttctagagtatgcacatggtgatgatgtgttgggttgataaagcactggctcagtcctacaggcactaaacttcaatggatactttgttaactatagttacactaactttaaagaaagttcttgatacctgttctttattcttaggaactgaagaggagggaactccggtgtttgcataatcatcgccttcccatgttaagaggactcaccctagtaggcttaatgggttttgtatttggttggcttgttttcccaagagacactaaagttgttcttgcattaattccccttaaaattgccaagagataagaggtgggaagacaaaaagggcgcctgattctattcagtagatgagaaaatagatttacagaaggtaactgtgaaattggaggagtaatgtcagggaggccttgtcaggacaggcaatgtcaaggaagcctatcccttctttgtcagactccagaaaggattgagttcatctgttcttcacagatccactttcctaggcagatgccagtgccttccaggtttgtatgaaagcaaaaaactgctgacgatgggcagagggcctgtcccaaaccactaggaagcaggagagggcaggaatctcagtgaatcccagatgtatccacctgtgctgaaggctaacccccaacctgtttggtgatgtgtgagcagccagttggtttcatgggtcagaagagtgtggtaatggtacctggaatcctgcaaaatgcatggaaacaaggaagagcagatccttattccaacatgaacagcaggacttataaggaaagcaggcttttccccatgacctcacagctctgcctccacctttcatctcttcacagtgagctttctttcagagtgatcttaccacccaaccaggcacagtctaatttgatcataacaaggaggaggccgggcacagtggctcatgcctataatcccagcactttgggaggctgaggtgggtggatcacttaagcccaggagtttcagacgtacctgggcaacatggagaaaccctgtctctacaaaaattagctgggcacatggtggtctatgcttacagtcccagctactcagttggctcaggcaggaggattgcttgagcccgggaggcagagtttgcagtgagctgagattgtgccactgtaatacagcctgggaaacagagcaagatcctgtctcaaacaaaacaaaacaaaaaatcaccaaataaacgataaggaagtcaccctgtccaaggaatgccgtttcatatggtgccaccccttctcctagaccaaagttcccattttagaaataactccatgctaggcaaggttgtaacggaaaagaaaggctctacctccagcctcccagatcaccccatctctactggctctccagaacccagtggggctcatagctattcctaagccaggccacaattcctgccagcccatgactagatccaaagcccgtgcaacagcgagaggagcaggggccgggcggggggggggggggcgcggtgtgtgcctttaaagatccggattatggtctttagcctgggttcaactgtagcacaaccaaccaccacggacgaccaatgaccgctatgagacagttcttcctttcacacagcagcatcatttatctggtagtagcaagacagccgtatgactttttgttgttgttaaagaaaaataagttgtcaagatttgcctaccaataactttcctatgtcttggctttcatgtccagtgggctagtttccaactgtttgagactcagggtaatcccagaaacctgtgaagcatcggcacaaaggttgtagcgcagatgccaacagatgtgtaggtaacaaacttgtaaggcacttcaatctccagtctccgcctggcctccttgttcctggtgaccaccttgaaccatgagtataatacttgcagtgagagattttgtacaagctgacgaaccaagaggatcaacacaattcccactgcaaatttggtcagacccaaaactaacatgtaggtggtgagtggtgggatgttctgaataacagggagagattcagcgggcttggatacaagctggaagaaatggttgatccagaatcctatggtcactccagccccggcagccagaatggtggtggtgtccgcccgggttgggctgtagtaatcagaaacagggtaattgtaacacaggaagaatggcacaactatgacacacacggggaagagggggctggccgagtccaggcagtcgatgaaggtccaggcagggtaggtgaggacgatgaggagtgcggtgatcaggacgccacccagcacatccaggaccgtatgcatcccagtgtagagcctgctgagacacaccaaggtggaaaacaccacggccatcaccagtcccaacacaaatggatactggtatctgtccatagtagagataaggagggtgaaggcaatggcagtggccgccatggcgtgggtggatggcattccatattcagcgatcagtctcttttccagttttacaactggaggggaggagggacggggccacttcaagacatccttggccacttggccaatatacatcaccaaaacccatatgatgatcaatcttctggataaataagggtcaatattccagtgagtgaatggaagaaacgtgatgtagaacacttcttggcccaaagcagctgaaaattggaataggtaatagtagaaataattcttcacgacgtacttctgtacataagcctccggcgccgcggctctgcgcagcccgttggccggagcctcgccgcccttgccgttggctgcggggagatgctcgaccccggggacccgcgccgcgcgctccgtggggtccgcgccgttctcccgggggccttcatccggagcggggaagagcccgcagcggcgctggaagcgggcgacgagctgggaatcctgcaggctccgcagcagctcggccatggtgtgcccggggccgcgctccgccgccgctgccacgccgggccggtgccctccgctggc

SEQ ID NO: 14044 - RNA, 3034 nt, Homo sapiens
  source 1..3034: mol_type = other RNA
gctgggattacaggcatgagccaccgcacccggcctaaaaattcttgagaaattggaatgctaagttacatactaaatatcatcccaacagtaaggccgtagaacatatttgaaatcaagaaaaatgtgatttttcggttttaacacgttaagagcctctgtaacttttaaggaagctatttttttttctagagtatgcacatggtgatgatgtgttgggttgataaagcactggctcagtcctacaggcactaaacttcaatggatactttgttaactatagttacactaactttaaagaaagttcttgatacctgttctttattcttaggaactgaagaggagggaactccggtgtttgcataatcatcgccttcccatgttaagaggactcaccctagtaggcttaatgggttttgtatttggttggcttgttttcccaagagacactaaagttgttcttgcattaattccccttaaaattgccaagagataagaggtgggaagacaaaaagggcgcctgattctattcagtagatgagaaaatagatttacagaaggtaactgtgaaattggaggagtaatgtcagggaggccttgtcaggacaggcaatgtcaaggaagcctatcccttctttgtcagactccagaaaggattgagttcatctgttcttcacagatccactttcctaggcagatgccagtgccttccaggtttgtatgaaagcaaaaaactgctgacgatgggcagagggcctgtcccaaaccactaggaagcaggagagggcaggaatctcagtgaatcccagatgtatccacctgtgctgaaggctaacccccaacctgtttggtgatgtgtgagcagccagttggtttcatgggtcagaagagtgtggtaatggtacctggaatcctgcaaaatgcatggaaacaaggaagagcagatccttattccaacatgaacagcaggacttataaggaaagcaggcttttccccatgacctcacagctctgcctccacctttcatctcttcacagtgagctttctttcagagtgatcttaccacccaaccaggcacagtctaatttgatcataacaaggaggaggccgggcacagtggctcatgcctataatcccagcactttgggaggctgaggtgggtggatcacttaagcccaggagtttcagacgtacctgggcaacatggagaaaccctgtctctacaaaaattagctgggcacatggtggtctatgcttacagtcccagctactcagttggctcaggcaggaggattgcttgagcccgggaggcagagtttgcagtgagctgagattgtgccactgtaatacagcctgggaaacagagcaagatcctgtctcaaacaaaacaaaacaaaaaatcaccaaataaacgataaggaagtcaccctgtccaaggaatgccgtttcatatggtgccaccccttctcctagaccaaagttcccattttagaaataactccatgctaggcaaggttgtaacggaaaagaaaggctctacctccagcctcccagatcaccccatctctactggctctccagaacccagtggggctcatagctattcctaagccaggccacaattcctgccagcccatgactagatccaaagcccgtgcaacagcgagaggagcaggggccgggcggggggggggggggcgcggtgtgtgcctttaaagatccggattatggtctttagcctgggttcaactgtagcacaaccaaccaccacggacgaccaatgaccgctatgagacagttcttcctttcacacagcagcatcatttatctggtagtagcaagacagccgtatgactttttgttgttgttaaagaaaaataagttgtcaagatttgcctaccaataactttcctatgtcttggctttcatgtccagtgggctagtttccaactgtttgagactcagggtaatcccagaaacctgtgaagcatcggcacaaaggttgtagcgcagatgccaacagatgtgtaggtaacaaacttgtaaggcacttcaatctccagtctccgcctggcctccttgttcctggtgaccaccttgaaccatgagtataatacttgcagtgagagattttgtacaagctgacgaaccaagaggatcaacacaattcccactgcaaatttggtcagacccaaaactaacatgtaggtggtgagtggtgggatgttctgaataacagggagagattcagcgggcttggatacaagctggaagaaatggttgatccagaatcctatggtcactccagccccggcagccagaatggtggtggtgtccgcccgggttgggctgtagtaatcagaaacagggtaattgtaacacaggaagaatggcacaactatgacacacacggggaagagggggctggccgagtccaggcagtcgatgaaggtccaggcagggtaggtgaggacgatgaggagtgcggtgatcaggacgccacccagcacatccaggaccgtatgcatcccagtgtagagcctgctgagacacaccaaggtggaaaacaccacggccatcaccagtcccaacacaaatggatactggtatctgtccatagtagagataaggagggtgaaggcaatggcagtggccgccatggcgtgggtggatggcattccatattcagcgatcagtctcttttccagttttacaactggaggggaggagggacggggccacttcaagacatccttggccacttggccaatatacatcaccaaaacccatatgatgatcaatcttctggataaataagggtcaatattccagtgagtgaatggaagaaacgtgatgtagaacacttcttggcccaaagcagctgaaaattggaataggtaatagtagaaataattcttcacgacgtacttctgtacataagccttcctgcaagactagttcccagtaaatacagcgagccccccagggagaattcccaagttctttccaaactgcgtgatgcaacgtctccct

SEQ ID NO: 14045 - RNA, 5034 nt, Homo sapiens
  source 1..5034: mol_type = other RNA
gctgggattacaggcatgagccaccgcacccggcctatattctaaattcttaaggtacttcaacttctcttggcattcagtctaaacaatgagtgcactgaaaagcctactatctgttaattatttctctactcaagtacagcacaagaggccttaggcaaacgaggggagccgaaagctttttatgcagacctctaaagtcagtgtactctgcctttgatttctttgattttatttacaagcttccatcccttctcagaaaataataaccaaaaaaataaaactggcacagtgaagtacattctcctcccattacatgaactagttcctaacagttacaggcaagaggttgcagatgaagaactgacttcccatcggtttcccttgtaacttctccagagactcatctatacgggaaatccagtcatctcaaactcaaaatgtcacaaagaaaaaacttgtatcattcggctggcccccagccactgtctcaaaccaggttctgctgaaagttgttccagcttttgttacaaatactgcagagtcactgaaaaaagttctaatcatacaaaggtctcatagttctacacattcaagagttgaaataagaaggaaatcttatatatgagctgaaaaaagagtaccccacaagctatttattagcatcaacattggaggtggtttgtatgactattcctccacgtaacactataccattctttatttaaaaagcaaatggtcagaacctttaggaaaaagcctttattaagaaactgcttgatatggtttggctgtgtttccacccaaatctcatcttgaattgtagttcccacaattcccatgtgttgtgggagggaccaggtaggaggtaattgaatcatggaggagggcctttcctgtgctgttcttgagatagtgaataaatctcacaagatctgatggttttacgaaggggggtttccctgcacaagttctcttctcttgtctgcctccatgtgagacgtgactttcaccttccgccacgattgtgatgccaccccagccacgtgaactgtgagtccattaaacctcttttttcttataaattacccaatctcaggtatgtctttatcagcagcgtgagaaaagactaatacactgctataggcaaggcacaattctagatgctttttatacttcacttcatttagccgtcacaatcaccccagaaaacagagctactcccacattgcagttaagaatgagaaactgtgaaacgaggattagaaaacacattcaccagtgcaaagttcagcggcccgcaagaccacctccagatttaacagttcactagaaggacccacagaactctctgaaagctgttatattcatgtatgttttattatagcataaggacacacattaacgctaaccgagggaacaggcacgtgggaccgagtctaggagaattccatgcctggagcttccggttgtcctatcgcagaggggttatagacagagctaacttctcccagcagggatgtgtgatgatatgcacagagtgctgccaaccttggaaatgcacctgagtcttggtgtccaaagattttactgcagctcagtcacctagacacagttgactgctacatgtctgaccttaatttccagcccctccagaggttgagccaataactgcatggcccaaagccccaactatatgaaaccatttggttggcagagaatatctggtgtgggggccgggtttggtggctcacgcctgtaatcccagcactttgggcagctgaggtgggaggatcacctgaggtcaggagtttgagaccagcctggccaacatggtgaaactccgtctctactaaaaatacaaaaattagccgggtgtggtggtgcatgcctgtaatcccagctacgtaggaggctgaggcaggagaatcaattgaacctgggaggcggaggttgctgtgagcagagatcgtgccactgcattccagcatgggcgacagagtgagacgcccatctcaaaaaaataataataataatagaatatctggtgtggcctaaggcctacaaataaacaaaggtactcttatcaggcaggacattccaagggcttggaggtcacctcccagaagctgagggcaaaggtcagccctttgtttgggtaaaattcatctatctgcacaatcagcatttcaaaggccatatataatagacaaaacggaataaaacaaaaataaaaaagaacactaatgcaaaacgaatcattcatattattttcatttctacactcaagggcttttatgtgatcttagtgtcaattattattttctaaatgggtcttccaaacatacaatcatacttacaagccacacagcaggggaagtattgatgaaagaagagaggctaccggaccttctcacaactcaaaattaatgttaactgtgtgggagtagaggaagtccaggggtcgtctgagggagaagtgattttggaatactgaggggtgatttttagactacaaaaaagagtattactgaaaccacccagtgggttcaccttgcccactgcctagacagagccaattaatcaagacaggggaactgtaatggagaaagagtaattcacacagagccagctgtgcgggagactggagttttatgattactcaaatcggtgtccctgaacattcaagcagcagagtttttaaggacaacttggtgggttgggggaagccagtgagccaggagtgctgattggtcagagatgacatcactgggaactgaagatgtcctcttgagctgagtcagttcctgggtggtggccacaagatcagatgagccagtttatcgagctgggtggtgccagctgatccatcaagtgcaaggtctgcaaaatttctcaagcactcatcctttctgtgtgctatcaggaggcaattagagtgttcgtgttcacatgcaatttcatattcggggatcagatccaccaactcgtggacaaactgtaccacttcctcatgccagggcacgtgggccatggtaagactgcttgctgaactttctccgcagtaggtaacgcccttcacttcgatgaagtcaggattccccagggacacgagctgcgcgtaggcctggagctcgtccacgttccatgctttcacgagcgtcagtctgtagacagttcgttgttgcttgactgccaaggcttttaaactgtcaaggaatctctgccagaaatccttgaagagtgggcggtcgattttcttcaggctgtctttggtactggcatccacactgacatacagctgagtaaccggctcgaggttcctgatttccgcaggaaattgtgcgtttgtgaccaggaagctggaaattttacactggtggagtagcttcaaaaacctgttgatctctgggtacattattggttctcccacgagggacaatgcacagtgctttaccgtcattccttcttcaaagcgttctgctttgacgcccggtactcctttaaactgcttaatcatgttctgatggttttcaatggcttccttcaagatcatttcaggctggtccatcttccaccgccactcagtgcccacggggttggtgtggtgccgccaacagaagacacatttattagcacacgccaagctcggggtggtttccatgcagcgatggctctcaattccatagaatgtgtgtttgtaacaacctcctctccctcggagcatggactttgtccacctgcaaagcttcacccccgagtggctcccaatcaactgataaccttgtttagtaagggcttctcggagagcaggagttatcatagctcttctttcaccatcttcattcctccccatgttcctgaacaaaccagacttctcttcctgctgttccttttctctcttttctttcttcacatgatccataattttgcccaaatcttcaacatcaacaatggaatttaggctctgatggtcctcaccaccaaactcttcttcactggagctctcaaagggttcttcctcctcggtgtctctatgatgcaattcatcctgctcatgagatccttcctccctctcctctgagccatgttggtgagattcacatttgcctttcttgcagtggccgccacaggacttctttctctcccctttctgaagtgcctgcagctgggagatgaacttggtcttccatgctctgaagtcggcctcaatgctgccgtgcttgcttttaaccacgtcgcagtcgccctcccctcgactcatcacacgatgcgcgccaagcatccagagccacttgtcaacatttttgccaaccttgttgaagtggctagcataggcagaatttcccaggccaaataccgcatatctcatacccttcaggtaagttttgccaaatcgaaaatcaatggatgcttcctctaaccatttgcagaaccactctgcactttcagttggtaggccgtcagtgtatgtcgcaaccaggaagacacagacatttttactagtcacctcttctatcagatgatcatctggatcatattcttttagattaataatggccacaggcagatccagggatgtaactgcttcagcaagaactgttgcgaatcccttcgctgttccagtctgagaaccataaaaaatcttcactccagacacaaagatgtctttctcttgaagggagacataaccatttgtcatcaaatcctgagctgcttttggaacagatttttcctgtaagttcttgccctgcgtcttgatgacaatctggacacaaatccaaaggctaatgctaacagcaaagcccaaataaatgtaaaacctgtttatccataatgatattaaaggtgagaagaggtcccatgtatccgcagaaggatccatcctcctcagagccgacaggagactaggatctcggacctggatagcccgatgattcgcactggtaccgcgagacgcaccgagctacctcgccgcgttagcggcgtaccgagtgcctgcagacctgtgggcagccatgacactgccaggcc

SEQ ID NO: 14046 - RNA, 1468 nt, Homo sapiens
  source 1..1468: mol_type = other RNA
gctgggattacaggcatgagccaccgcacccggcctcacttcaagaattttttacaagcacagaaactatatctcagtgtatgataactgttactataatactatattgtattataaatatacaagctcatttgagtgtgtgatagctccactacctccaccaagctttaggaatatatataatctactttgaacccaaaagccacagaagcagtgacaacgacgctaagaagcagaaagagtatatggttagtagaaactatctggcatcttgctcacctgaactacacctaaagtgctgttatttcccgtacatgcacttttccattatgttcttcacaaaggctcacctcttttccataagccaccatgcccagtccacaaaccaaattatttttaatgttcaacagaaaagaaaggtagcaacaagttccttatttttgttaattccttgtttcttgtaataaagagtatcacttcctctcaccaaaaagctatagagcttctgatgaaattcaactgttcaaaaggtttacctcttttccaggggtaggtgtgattaaacagctggcatttcttcttaacaaagtaatgaaaaggcaattactaaaaaatcagcattgtattaccagaaaggcaagtcatttcataaaataagaactggagagttttaaatccatattcattaagaagctaaaaaattcatactaatttttaaccacttagagttttgactcacaataatcaaaccactttccagtttataaataattcaagatcaaaataataaattttaaaattaagcaaaatttgaaaaacttacatataaatatcaaaaaccatgcaacatgacgtctgctacttggaaaaaaggcatggagacacagtaataccggaataaggatttcaacatatgacataatggcataaggcactacctcaacttcagtctacacttgagtcatcataacccaaatatgggacaggagaagaaaacacacaaacacaacttttcacatccttttggctggtctggcagttaactgcttttctctttcaaactccttctctcgttgctgctccctttccaactcttctttttgcctcttctgctgcagtttaagtgctcttttcaaagcattaatatccaacatagaatgacattctttaaattttgaaatctcttgttccagtgtgtctaacaatacaacttggttctgtgtgagttcctggagggcttgttttgatctctgcagatctggcaaataatgagaaagcaatccttctgccagttgctccactgctttgtcttctatagtcaagtcctctattaacccttcatctggagaagtgtcacttaaacctctctgaattataagctgatcatctttctggtaaatccatcccccaccactgccgtatgacaaataaccaatgacgtaccggagtcaacacataaactcagaat

SEQ ID NO: 14047 - RNA, 1707 nt, Homo sapiens
  source 1..1707: mol_type = other RNA
gctgggattacaggcatgagccaccgcacccggcctcacttcaagaattttttacaagcacagaaactatatctcagtgtatgataactgttactataatactatattgtattataaatatacaagctcatttgagtgtgtgatagctccactacctccaccaagctttaggaatatatataatctactttgaacccaaaagccacagaagcagtgacaacgacgctaagaagcagaaagagtatatggttagtagaaactatctggcatcttgctcacctgaactacacctaaagtgctgttatttcccgtacatgcacttttccattatgttcttcacaaaggctcacctcttttccataagccaccatgcccagtccacaaaccaaattatttttaatgttcaacagaaaagaaaggtagcaacaagttccttatttttgttaattccttgtttcttgtaataaagagtatcacttcctctcaccaaaaagctatagagcttctgatgaaattcaactgttcaaaaggtttacctcttttccaggggtaggtgtgattaaacagctggcatttcttcttaacaaagtaatgaaaaggcaattactaaaaaatcagcattgtattaccagaaaggcaagtcatttcataaaataagaactggagagttttaaatccatattcattaagaagctaaaaaattcatactaatttttaaccacttagagttttgactcacaataatcaaaccactttccagtttataaataattcaagatcaaaataataaattttaaaattaagcaaaatttgaaaaacttacatataaatatcaaaaaccatgcaacatgacgtctgctacttggaaaaaaggcatggagacacagtaataccggaataaggatttcaacatatgacataatggcataaggcactacctcaacttcagtctacacttgagtcatcataacccaaatatgggacaggagaagaaaacacacaaacacaacttttcacatccttttggctggtctggcagttaactgcttttctctttcaaactccttctctcgttgctgctccctttccaactcttctttttgcctcttctgctgcagtttaagtgctcttttttttaactttgatgttttttcatgaagcatcagcatctcttttcttatattcaccaacttggcatgatagtgtttagcctcagcaaacaaagcattaatatccaacatagaatgacattctttaaattttgaaatctcttgttccagtgtgtctaacaatacaacttggttcaggcgtcggctccccggcctccaggcagtagggtggccgtgtcagggccccgtccggagacgacggcccagggacactcatgtccctccagctgggaacacagggaagaagcaaacgtgtggctcgtcagaagcaaggcggcacctaacgactccagcggctggccggacagaagagattgtcgcacccggaagtgacgggggcgaaaaaactgcgggcttcgatcacgcgctcgagagttggctctgccccatggcgttgtggggaccccgcgctgatatcgtcgtctggccccggacgcagtgtcagcggactcagcagtgtggggctcgagtccctgcgatccgattggtgggagctgggggaggacggtggtcggtttgggctgctcacggggtgggt

SEQ ID NO: 14048 - RNA, 1711 nt, Homo sapiens
  source 1..1711: mol_type = other RNA
gctgggattacaggcatgagccaccgcacccggcctcacttcaagaattttttacaagcacagaaactatatctcagtgtatgataactgttactataatactatattgtattataaatatacaagctcatttgagtgtgtgatagctccactacctccaccaagctttaggaatatatataatctactttgaacccaaaagccacagaagcagtgacaacgacgctaagaagcagaaagagtatatggttagtagaaactatctggcatcttgctcacctgaactacacctaaagtgctgttatttcccgtacatgcacttttccattatgttcttcacaaaggctcacctcttttccataagccaccatgcccagtccacaaaccaaattatttttaatgttcaacagaaaagaaaggtagcaacaagttccttatttttgttaattccttgtttcttgtaataaagagtatcacttcctctcaccaaaaagctatagagcttctgatgaaattcaactgttcaaaaggtttacctcttttccaggggtaggtgtgattaaacagctggcatttcttcttaacaaagtaatgaaaaggcaattactaaaaaatcagcattgtattaccagaaaggcaagtcatttcataaaataagaactggagagttttaaatccatattcattaagaagctaaaaaattcatactaatttttaaccacttagagttttgactcacaataatcaaaccactttccagtttataaataattcaagatcaaaataataaattttaaaattaagcaaaatttgaaaaacttacatataaatatcaaaaaccatgcaacatgacgtctgctacttggaaaaaaggcatggagacacagtaataccggaataaggatttcaacatatgacataatggcataaggcactacctcaacttcagtctacacttgagtcatcataacccaaatatgggacaggagaagaaaacacacaaacacaacttttcacatccttttggctggtctggcagttaactgcttttctctttcaaactccttctctcgttgctgctccctttccaactcttctttttgcctcttctgctgcagtttaagtgctcttttttttaactttgatgttttttcatgaagcatcagcatctcttttcttatattcaccaacttggcatgatagtgtttagcctcagcaaacaaagcattaatatccaacatagaatgacattctttaaattttgaaatctcttgttccagtgtgtctaacaatacaacttggttctgtcaggcgtcggctccccggcctccaggcagtagggtggccgtgtcagggccccgtccggagacgacggcccagggacactcatgtccctccagctgggaacacagggaagaagcaaacgtgtggctcgtcagaagcaaggcggcacctaacgactccagcggctggccggacagaagagattgtcgcacccggaagtgacgggggcgaaaaaactgcgggcttcgatcacgcgctcgagagttggctctgccccatggcgttgtggggaccccgcgctgatatcgtcgtctggccccggacgcagtgtcagcggactcagcagtgtggggctcgagtccctgcgatccgattggtgggagctgggggaggacggtggtcggtttgggctgctcacggggtgggt

SEQ ID NO: 14049 - RNA, 1861 nt, Homo sapiens
  source 1..1861: mol_type = other RNA
gctgggattacaggcatgagccaccgcacccggcctcacttcaagaattttttacaagcacagaaactatatctcagtgtatgataactgttactataatactatattgtattataaatatacaagctcatttgagtgtgtgatagctccactacctccaccaagctttaggaatatatataatctactttgaacccaaaagccacagaagcagtgacaacgacgctaagaagcagaaagagtatatggttagtagaaactatctggcatcttgctcacctgaactacacctaaagtgctgttatttcccgtacatgcacttttccattatgttcttcacaaaggctcacctcttttccataagccaccatgcccagtccacaaaccaaattatttttaatgttcaacagaaaagaaaggtagcaacaagttccttatttttgttaattccttgtttcttgtaataaagagtatcacttcctctcaccaaaaagctatagagcttctgatgaaattcaactgttcaaaaggtttacctcttttccaggggtaggtgtgattaaacagctggcatttcttcttaacaaagtaatgaaaaggcaattactaaaaaatcagcattgtattaccagaaaggcaagtcatttcataaaataagaactggagagttttaaatccatattcattaagaagctaaaaaattcatactaatttttaaccacttagagttttgactcacaataatcaaaccactttccagtttataaataattcaagatcaaaataataaattttaaaattaagcaaaatttgaaaaacttacatataaatatcaaaaaccatgcaacatgacgtctgctacttggaaaaaaggcatggagacacagtaataccggaataaggatttcaacatatgacataatggcataaggcactacctcaacttcagtctacacttgagtcatcataacccaaatatgggacaggagaagaaaacacacaaacacaacttttcacatccttttggctggtctggcagttaactgcttttctctttcaaactccttctctcgttgctgctccctttccaactcttctttttgcctcttctgctgcagtttaagtgctcttttttttaactttgatgttttttcatgaagcatcagcatctcttttcttatattcaccaacttggcatgatagtgtttagcctcagcaaacaaagcattaatatccaacatagaatgacattctttaaattttgaaatctcttgttccagtgtgtctaacaatacaacttggttctgtcttccaaaaaagacagtaccgggaccaaacggcttcactggtaatttttaccaaacatttaaggaagacgtgataccaattccccacagtctcttccagaaaatatgtcagtcctcctttatctgcagttttgctttcttcagttttaggcacgtacagtcaactgcagctgtggtgagttcctggagggcttgttttgatctctgcagatctggcaaataatgagaaagcaatccttctgccagttgctccactgctttgtcttctatagtcaagtcctctattaacccttcatctggagaagtgtcacttaaaccggagtcaacacataaactcagaatggcttcaccatcaaccgccttcaattgcacccccaatacaaagcttcccctcgggacttcagttccgcccattgcgctgggcagaggggccggcgcggttccccatttctgcactcggggcagggcccgggggccgcagccgccaaaaaccgcttactcccccagggtttctccggagttctactcactcaggtccccgcccctcacaccca

SEQ ID NO: 14050 - RNA, 1597 nt, Homo sapiens
  source 1..1597: mol_type = other RNA
gctgggattacaggcatgagccaccgcacccggcctcacttcaagaattttttacaagcacagaaactatatctcagtgtatgataactgttactataatactatattgtattataaatatacaagctcatttgagtgtgtgatagctccactacctccaccaagctttaggaatatatataatctactttgaacccaaaagccacagaagcagtgacaacgacgctaagaagcagaaagagtatatggttagtagaaactatctggcatcttgctcacctgaactacacctaaagtgctgttatttcccgtacatgcacttttccattatgttcttcacaaaggctcacctcttttccataagccaccatgcccagtccacaaaccaaattatttttaatgttcaacagaaaagaaaggtagcaacaagttccttatttttgttaattccttgtttcttgtaataaagagtatcacttcctctcaccaaaaagctatagagcttctgatgaaattcaactgttcaaaaggtttacctcttttccaggggtaggtgtgattaaacagctggcatttcttcttaacaaagtaatgaaaaggcaattactaaaaaatcagcattgtattaccagaaaggcaagtcatttcataaaataagaactggagagttttaaatccatattcattaagaagctaaaaaattcatactaatttttaaccacttagagttttgactcacaataatcaaaccactttccagtttataaataattcaagatcaaaataataaattttaaaattaagcaaaatttgaaaaacttacatataaatatcaaaaaccatgcaacatgacgtctgctacttggaaaaaaggcatggagacacagtaataccggaataaggatttcaacatatgacataatggcataaggcactacctcaacttcagtctacacttgagtcatcataacccaaatatgggacaggagaagaaaacacacaaacacaacttttcacatccttttggctggtctggcagttaactgcttttctctttcaaactccttctctcgttgctgctccctttccaactcttctttttgcctcttctgctgcagtttaagtgctcttttttttaactttgatgttttttcatgaagcatcagcatctcttttcttatattcaccaacttggcatgatagtgtttagcctcagcaaacaaagcattaatatccaacatagaatgacattctttaaattttgaaatctcttgttccagtgtgtctaacaatacaacttggttctgtgtgagttcctggagggcttgttttgatctctgcagatctggcaaataatgagaaagcaatccttctgccagttgctccactgctttgtcttctatagtcaagtcctctattaacccttcatctggagaagtgtcacttaaaccaggcgtcggctccccggcctccaggcagtagggtggccgtgtcagggccccgtccggagacgacggcccagggacactcatgtccctccagctgggaacacagggaagaagcaaacgtgtggctcgtcagaagcaaggcggcacct

SEQ ID NO: 14051 - RNA, 1687 nt, Homo sapiens
  source 1..1687: mol_type = other RNA
gctgggattacaggcatgagccaccgcacccggcctcacttcaagaattttttacaagcacagaaactatatctcagtgtatgataactgttactataatactatattgtattataaatatacaagctcatttgagtgtgtgatagctccactacctccaccaagctttaggaatatatataatctactttgaacccaaaagccacagaagcagtgacaacgacgctaagaagcagaaagagtatatggttagtagaaactatctggcatcttgctcacctgaactacacctaaagtgctgttatttcccgtacatgcacttttccattatgttcttcacaaaggctcacctcttttccataagccaccatgcccagtccacaaaccaaattatttttaatgttcaacagaaaagaaaggtagcaacaagttccttatttttgttaattccttgtttcttgtaataaagagtatcacttcctctcaccaaaaagctatagagcttctgatgaaattcaactgttcaaaaggtttacctcttttccaggggtaggtgtgattaaacagctggcatttcttcttaacaaagtaatgaaaaggcaattactaaaaaatcagcattgtattaccagaaaggcaagtcatttcataaaataagaactggagagttttaaatccatattcattaagaagctaaaaaattcatactaatttttaaccacttagagttttgactcacaataatcaaaccactttccagtttataaataattcaagatcaaaataataaattttaaaattaagcaaaatttgaaaaacttacatataaatatcaaaaaccatgcaacatgacgtctgctacttggaaaaaaggcatggagacacagtaataccggaataaggatttcaacatatgacataatggcataaggcactacctcaacttcagtctacacttgagtcatcataacccaaatatgggacaggagaagaaaacacacaaacacaacttttcacatccttttggctggtctggcagttaactgcttttctctttcaaactccttctctcgttgctgctccctttccaactcttctttttgcctcttctgctgcagtttaagtgctcttttttttaactttgatgttttttcatgaagcatcagcatctcttttcttatattcaccaacttggcatgatagtgtttagcctcagcaaacaaagcattaatatccaacatagaatgacattctttaaattttgaaatctcttgttccagtgtgtctaacaatacaacttggttctgtgtgagttcctggagggcttgttttgatctctgcagatctggcaaataatgagaaagcaatccttctgccagttgctccactgctttgtcttctatagtcaagtcctctattaacccttcatctggagaagtgtcacttaaaccggagtcaacacataaactcagaatggcttcaccatcaaccgccttcaattgcacccccaatacaaagcttcccctcgggacttcagttccgcccattgcgctgggcagaggggccggcgcggttccccatttctgcactcggggcagggcccgggggccgcagccgccaaaaaccgcttactcccccagggtttctccggagttctactcactcaggtccccgcccctcacaccca

SEQ ID NO: 14052 - RNA, 1555 nt, Homo sapiens
  source 1..1555: mol_type = other RNA
gctgggattacaggcatgagccaccgcacccggcctcacttcaagaattttttacaagcacagaaactatatctcagtgtatgataactgttactataatactatattgtattataaatatacaagctcatttgagtgtgtgatagctccactacctccaccaagctttaggaatatatataatctactttgaacccaaaagccacagaagcagtgacaacgacgctaagaagcagaaagagtatatggttagtagaaactatctggcatcttgctcacctgaactacacctaaagtgctgttatttcccgtacatgcacttttccattatgttcttcacaaaggctcacctcttttccataagccaccatgcccagtccacaaaccaaattatttttaatgttcaacagaaaagaaaggtagcaacaagttccttatttttgttaattccttgtttcttgtaataaagagtatcacttcctctcaccaaaaagctatagagcttctgatgaaattcaactgttcaaaaggtttacctcttttccaggggtaggtgtgattaaacagctggcatttcttcttaacaaagtaatgaaaaggcaattactaaaaaatcagcattgtattaccagaaaggcaagtcatttcataaaataagaactggagagttttaaatccatattcattaagaagctaaaaaattcatactaatttttaaccacttagagttttgactcacaataatcaaaccactttccagtttataaataattcaagatcaaaataataaattttaaaattaagcaaaatttgaaaaacttacatataaatatcaaaaaccatgcaacatgacgtctgctacttggaaaaaaggcatggagacacagtaataccggaataaggatttcaacatatgacataatggcataaggcactacctcaacttcagtctacacttgagtcatcataacccaaatatgggacaggagaagaaaacacacaaacacaacttttcacatccttttggctggtctggcagttaactgcttttctctttcaaactccttctctcgttgctgctccctttccaactcttctttttgcctcttctgctgcagtttaagtgctcttttttttaactttgatgttttttcatgaagcatcagcatctcttttcttatattcaccaacttggcatgatagtgtttagcctcagcaaacaaagcattaatatccaacatagaatgacattctttaaattttgaaatctcttgttccagtgtgtctaacaatacaacttggttctgtgtgagttcctggagggcttgttttgatctctgcagatctggcaaataatgagaaagcaatccttctgccagttgctccactgctttgtcttctatagtcaagtcctctattaacccttcatctggagaagtgtcacttaaacctctctgaattataagctgatcatctttctggtaaatccatcccccaccactgccgtatgacaaataaccaatgacgtaccggagtcaacacataaactcagaat

SEQ ID NO: 14053 - RNA, 1593 nt, Homo sapiens
  source 1..1593: mol_type = other RNA
gctgggattacaggcatgagccaccgcacccggcctcacttcaagaattttttacaagcacagaaactatatctcagtgtatgataactgttactataatactatattgtattataaatatacaagctcatttgagtgtgtgatagctccactacctccaccaagctttaggaatatatataatctactttgaacccaaaagccacagaagcagtgacaacgacgctaagaagcagaaagagtatatggttagtagaaactatctggcatcttgctcacctgaactacacctaaagtgctgttatttcccgtacatgcacttttccattatgttcttcacaaaggctcacctcttttccataagccaccatgcccagtccacaaaccaaattatttttaatgttcaacagaaaagaaaggtagcaacaagttccttatttttgttaattccttgtttcttgtaataaagagtatcacttcctctcaccaaaaagctatagagcttctgatgaaattcaactgttcaaaaggtttacctcttttccaggggtaggtgtgattaaacagctggcatttcttcttaacaaagtaatgaaaaggcaattactaaaaaatcagcattgtattaccagaaaggcaagtcatttcataaaataagaactggagagttttaaatccatattcattaagaagctaaaaaattcatactaatttttaaccacttagagttttgactcacaataatcaaaccactttccagtttataaataattcaagatcaaaataataaattttaaaattaagcaaaatttgaaaaacttacatataaatatcaaaaaccatgcaacatgacgtctgctacttggaaaaaaggcatggagacacagtaataccggaataaggatttcaacatatgacataatggcataaggcactacctcaacttcagtctacacttgagtcatcataacccaaatatgggacaggagaagaaaacacacaaacacaacttttcacatccttttggctggtctggcagttaactgcttttctctttcaaactccttctctcgttgctgctccctttccaactcttctttttgcctcttctgctgcagtttaagtgctcttttttttaactttgatgttttttcatgaagcatcagcatctcttttcttatattcaccaacttggcatgatagtgtttagcctcagcaaacaaagcattaatatccaacatagaatgacattctttaaattttgaaatctcttgttccagtgtgtctaacaatacaacttggttgtgagttcctggagggcttgttttgatctctgcagatctggcaaataatgagaaagcaatccttctgccagttgctccactgctttgtcttctatagtcaagtcctctattaacccttcatctggagaagtgtcacttaaaccaggcgtcggctccccggcctccaggcagtagggtggccgtgtcagggccccgtccggagacgacggcccagggacactcatgtccctccagctgggaacacagggaagaagcaaacgtgtggctcgtcagaagcaaggcggcacct

SEQ ID NO: 14054 - RNA, 1367 nt, Homo sapiens
  source 1..1367: mol_type = other RNA
gctgggattacaggcatgagccaccgcacccggcctcacttcaagaattttttacaagcacagaaactatatctcagtgtatgataactgttactataatactatattgtattataaatatacaagctcatttgagtgtgtgatagctccactacctccaccaagctttaggaatatatataatctactttgaacccaaaagccacagaagcagtgacaacgacgctaagaagcagaaagagtatatggttagtagaaactatctggcatcttgctcacctgaactacacctaaagtgctgttatttcccgtacatgcacttttccattatgttcttcacaaaggctcacctcttttccataagccaccatgcccagtccacaaaccaaattatttttaatgttcaacagaaaagaaaggtagcaacaagttccttatttttgttaattccttgtttcttgtaataaagagtatcacttcctctcaccaaaaagctatagagcttctgatgaaattcaactgttcaaaaggtttacctcttttccaggggtaggtgtgattaaacagctggcatttcttcttaacaaagtaatgaaaaggcaattactaaaaaatcagcattgtattaccagaaaggcaagtcatttcataaaataagaactggagagttttaaatccatattcattaagaagctaaaaaattcatactaatttttaaccacttagagttttgactcacaataatcaaaccactttccagtttataaataattcaagatcaaaataataaattttaaaattaagcaaaatttgaaaaacttacatataaatatcaaaaaccatgcaacatgacgtctgctacttggaaaaaaggcatggagacacagtaataccggaataaggatttcaacatatgacataatggcataaggcactacctcaacttcagtctacacttgagtcatcataacccaaatatgggacaggagaagaaaacacacaaacacaacttttcacatccttttggctggtctggcagttaactgcttttctctttcaaactccttctctcgttgctgctccctttccaactcttctttttgcctcttctgctgcagtttaagtgctcttttttttaactttgatgttttttcatgaagcatcagcatctcttttcttatattcaccaacttggcatgatagtgtttagcctcagcaaacaggcgtcggctccccggcctccaggcagtagggtggccgtgtcagggccccgtccggagacgacggcccagggacactcatgtccctccagctgggaacacagggaagaagcaaacgtgtggctcgtcagaagcaaggcggcacct

SEQ ID NO: 14055 - RNA, 1457 nt, Homo sapiens
  source 1..1457: mol_type = other RNA
gctgggattacaggcatgagccaccgcacccggcctcacttcaagaattttttacaagcacagaaactatatctcagtgtatgataactgttactataatactatattgtattataaatatacaagctcatttgagtgtgtgatagctccactacctccaccaagctttaggaatatatataatctactttgaacccaaaagccacagaagcagtgacaacgacgctaagaagcagaaagagtatatggttagtagaaactatctggcatcttgctcacctgaactacacctaaagtgctgttatttcccgtacatgcacttttccattatgttcttcacaaaggctcacctcttttccataagccaccatgcccagtccacaaaccaaattatttttaatgttcaacagaaaagaaaggtagcaacaagttccttatttttgttaattccttgtttcttgtaataaagagtatcacttcctctcaccaaaaagctatagagcttctgatgaaattcaactgttcaaaaggtttacctcttttccaggggtaggtgtgattaaacagctggcatttcttcttaacaaagtaatgaaaaggcaattactaaaaaatcagcattgtattaccagaaaggcaagtcatttcataaaataagaactggagagttttaaatccatattcattaagaagctaaaaaattcatactaatttttaaccacttagagttttgactcacaataatcaaaccactttccagtttataaataattcaagatcaaaataataaattttaaaattaagcaaaatttgaaaaacttacatataaatatcaaaaaccatgcaacatgacgtctgctacttggaaaaaaggcatggagacacagtaataccggaataaggatttcaacatatgacataatggcataaggcactacctcaacttcagtctacacttgagtcatcataacccaaatatgggacaggagaagaaaacacacaaacacaacttttcacatccttttggctggtctggcagttaactgcttttctctttcaaactccttctctcgttgctgctccctttccaactcttctttttgcctcttctgctgcagtttaagtgctcttttttttaactttgatgttttttcatgaagcatcagcatctcttttcttatattcaccaacttggcatgatagtgtttagcctcagcaaacggagtcaacacataaactcagaatggcttcaccatcaaccgccttcaattgcacccccaatacaaagcttcccctcgggacttcagttccgcccattgcgctgggcagaggggccggcgcggttccccatttctgcactcggggcagggcccgggggccgcagccgccaaaaaccgcttactcccccagggtttctccggagttctactcactcaggtccccgcccctcacaccca

SEQ ID NO: 14056 - RNA, 1325 nt, Homo sapiens
  source 1..1325: mol_type = other RNA
gctgggattacaggcatgagccaccgcacccggcctcacttcaagaattttttacaagcacagaaactatatctcagtgtatgataactgttactataatactatattgtattataaatatacaagctcatttgagtgtgtgatagctccactacctccaccaagctttaggaatatatataatctactttgaacccaaaagccacagaagcagtgacaacgacgctaagaagcagaaagagtatatggttagtagaaactatctggcatcttgctcacctgaactacacctaaagtgctgttatttcccgtacatgcacttttccattatgttcttcacaaaggctcacctcttttccataagccaccatgcccagtccacaaaccaaattatttttaatgttcaacagaaaagaaaggtagcaacaagttccttatttttgttaattccttgtttcttgtaataaagagtatcacttcctctcaccaaaaagctatagagcttctgatgaaattcaactgttcaaaaggtttacctcttttccaggggtaggtgtgattaaacagctggcatttcttcttaacaaagtaatgaaaaggcaattactaaaaaatcagcattgtattaccagaaaggcaagtcatttcataaaataagaactggagagttttaaatccatattcattaagaagctaaaaaattcatactaatttttaaccacttagagttttgactcacaataatcaaaccactttccagtttataaataattcaagatcaaaataataaattttaaaattaagcaaaatttgaaaaacttacatataaatatcaaaaaccatgcaacatgacgtctgctacttggaaaaaaggcatggagacacagtaataccggaataaggatttcaacatatgacataatggcataaggcactacctcaacttcagtctacacttgagtcatcataacccaaatatgggacaggagaagaaaacacacaaacacaacttttcacatccttttggctggtctggcagttaactgcttttctctttcaaactccttctctcgttgctgctccctttccaactcttctttttgcctcttctgctgcagtttaagtgctcttttttttaactttgatgttttttcatgaagcatcagcatctcttttcttatattcaccaacttggcatgatagtgtttagcctcagcaaactctctgaattataagctgatcatctttctggtaaatccatcccccaccactgccgtatgacaaataaccaatgacgtaccggagtcaacacataaactcagaat

SEQ ID NO: 14057 - RNA, 1509 nt, Homo sapiens
  source 1..1509: mol_type = other RNA
gctgggattacaggcatgagccaccgcacccggcctcacttcaagaattttttacaagcacagaaactatatctcagtgtatgataactgttactataatactatattgtattataaatatacaagctcatttgagtgtgtgatagctccactacctccaccaagctttaggaatatatataatctactttgaacccaaaagccacagaagcagtgacaacgacgctaagaagcagaaagagtatatggttagtagaaactatctggcatcttgctcacctgaactacacctaaagtgctgttatttcccgtacatgcacttttccattatgttcttcacaaaggctcacctcttttccataagccaccatgcccagtccacaaaccaaattatttttaatgttcaacagaaaagaaaggtagcaacaagttccttatttttgttaattccttgtttcttgtaataaagagtatcacttcctctcaccaaaaagctatagagcttctgatgaaattcaactgttcaaaaggtttacctcttttccaggggtaggtgtgattaaacagctggcatttcttcttaacaaagtaatgaaaaggcaattactaaaaaatcagcattgtattaccagaaaggcaagtcatttcataaaataagaactggagagttttaaatccatattcattaagaagctaaaaaattcatactaatttttaaccacttagagttttgactcacaataatcaaaccactttccagtttataaataattcaagatcaaaataataaattttaaaattaagcaaaatttgaaaaacttacatataaatatcaaaaaccatgcaacatgacgtctgctacttggaaaaaaggcatggagacacagtaataccggaataaggatttcaacatatgacataatggcataaggcactacctcaacttcagtctacacttgagtcatcataacccaaatatgggacaggagaagaaaacacacaaacacaacttttcacatccttttggctggtctggcagttaactgcttttctctttcaaactccttctctcgttgctgctccctttccaactcttctttttgcctcttctgctgcagtttaagtgctcttttttttaactttgatgttttttcatgaagcatcagcatctcttttcttatattcaccaacttggcatgatagtgtttagcctcagcaaagtgagttcctggagggcttgttttgatctctgcagatctggcaaataatgagaaagcaatccttctgccagttgctccactgctttgtcttctatagtcaagtcctctattaacccttcatctggagaagtgtcacttaaaccaggcgtcggctccccggcctccaggcagtagggtggccgtgtcagggccccgtccggagacgacggcccagggacactcatgtccctccagctgggaacacagggaagaagcaaacgtgtggctcgtcagaagcaaggcggcacct

SEQ ID NO: 14058 - RNA, 1599 nt, Homo sapiens
  source 1..1599: mol_type = other RNA
gctgggattacaggcatgagccaccgcacccggcctcacttcaagaattttttacaagcacagaaactatatctcagtgtatgataactgttactataatactatattgtattataaatatacaagctcatttgagtgtgtgatagctccactacctccaccaagctttaggaatatatataatctactttgaacccaaaagccacagaagcagtgacaacgacgctaagaagcagaaagagtatatggttagtagaaactatctggcatcttgctcacctgaactacacctaaagtgctgttatttcccgtacatgcacttttccattatgttcttcacaaaggctcacctcttttccataagccaccatgcccagtccacaaaccaaattatttttaatgttcaacagaaaagaaaggtagcaacaagttccttatttttgttaattccttgtttcttgtaataaagagtatcacttcctctcaccaaaaagctatagagcttctgatgaaattcaactgttcaaaaggtttacctcttttccaggggtaggtgtgattaaacagctggcatttcttcttaacaaagtaatgaaaaggcaattactaaaaaatcagcattgtattaccagaaaggcaagtcatttcataaaataagaactggagagttttaaatccatattcattaagaagctaaaaaattcatactaatttttaaccacttagagttttgactcacaataatcaaaccactttccagtttataaataattcaagatcaaaataataaattttaaaattaagcaaaatttgaaaaacttacatataaatatcaaaaaccatgcaacatgacgtctgctacttggaaaaaaggcatggagacacagtaataccggaataaggatttcaacatatgacataatggcataaggcactacctcaacttcagtctacacttgagtcatcataacccaaatatgggacaggagaagaaaacacacaaacacaacttttcacatccttttggctggtctggcagttaactgcttttctctttcaaactccttctctcgttgctgctccctttccaactcttctttttgcctcttctgctgcagtttaagtgctcttttttttaactttgatgttttttcatgaagcatcagcatctcttttcttatattcaccaacttggcatgatagtgtttagcctcagcaaagtgagttcctggagggcttgttttgatctctgcagatctggcaaataatgagaaagcaatccttctgccagttgctccactgctttgtcttctatagtcaagtcctctattaacccttcatctggagaagtgtcacttaaaccggagtcaacacataaactcagaatggcttcaccatcaaccgccttcaattgcacccccaatacaaagcttcccctcgggacttcagttccgcccattgcgctgggcagaggggccggcgcggttccccatttctgcactcggggcagggcccgggggccgcagccgccaaaaaccgcttactcccccagggtttctccggagttctactcactcaggtccccgcccctcacaccca

SEQ ID NO: 14059 - RNA, 3271 nt, Homo sapiens
  source 1..3271: mol_type = other RNA
gctgggattacaggcatgagccaccgcacccggcctggcacacatttaatttaatttagcagtaacttactccctgcgcccagaagaggtaggggcaagagttgctttccatgaagagtgcacctgatgagaaggcagctccagaagactcaaaggaaaaccgagaatcaggagagaaagaaacgtgcagtccttgcctacttcaggggaggaccccaaactcccggttgatagtagggacctgcttccccatgcgccccagctccctctccaccatgcagtcgcctcctgggcctggcgaccacagttcggggcctgctctaaggcccagagttctcagtcaggcgatgcccagctgaagtggtctgggcctcgtggcagcaccagatccagggtgaggtcacgctgctggtccgcagagtacacaggccggtagcccagcagctgcagcgcgccggcgcacacctcctgcacgcgcaggatcttagtgaagggcaacgcgtggcgccaggcctgggagacgttgcgcgcattcctagacgaagtatggaaggcctcgattggcttgccgatccccgacccgtgggtgatgttgtggatccaggcctcgagctgtggcgtgagggtcaggccggtgaaggcgtagagtgcgcggatctctgccagcggctcccgcgccaggtcctcgaagcgcaccaggcggtagcggccgcgcaggaagggtggcggcttgagtgtggcggcctcggcgatgcgcacgtggctgcggcacacctcgcgaatcaggcgcaggtgagggtcggcctccacccacttgccgttggtgcccagcacgatgccgttgtcgcgtgccagtatcgggcccgccgcctcccgggagcgcagcacggcccgcgggtcgcgcaccaggtgcacgatgcgcaggttgagcgcggggtcgctgagcagcgggtagagcacctgcaggttgaagaagcgcacctccttgagcaccacgtggctgtaggagcggcaggcctcccgggccaggctgaatggctgccgcgtgcacagtgtcttgcatacgtcctgcttgctgatggtgcctcggggaaaggcgctgcaggcgggcggcgagcacagcgcgcggctcgttgcccagttgaaaaaggcggacaggtttcggctctgtggcatgtaggcatcaaacacgtccatgtcgcacaaaaagatagagcgcatcaggtcgcgcacggccatgtgcagcgttgccgcgctgccctgcgacagggtggtccacacatgccacgcgggctccatcaggtagaagacgtcggggtgctggctgaagagctggcccaagaaggatgagcccgagcgccacgaggacagcaccagcacgtgcacacgatcctcgccgccggctggggatgagggccctggccgggagatgatgaagagcaggaggcaggtggtctgtgccaggaggagcactgtcactgtcttgctggagaaccgtggcagccacatgcgggcggctgggggccttcgggtggagtgggcaactttagggacccgggccctcatgcccatcccatgccccaattactgcccagtgccctcagggatcagccctcagattcggctaccctacccattggacttcccaagactcccaaggtctcagtcgagcactttcccaggaatacggagtcaagacataggccagaatatagtctgtgctcacagcagaagtccagttgcagaataatgtgggatatcatcaaactgtctacctacccacccacccacctacttacatacctacaggctatctatctgtagagagaaatactatgtttcaaagagaactcctgtcttttgcttcaggatacctcttagagagacccttttaggttgtggagctaaaagggcttgatgggggcttcggtggatgtcagagcaccaccaggctcgccgaggttgaatcctggctctgccacttcctagcctatgatcttgcttatgaagatcacttaaatctctctgtgacggatcactttacccgtgtgtgaaagagggataattccggtacctggctcacaggatctggggggattggggggttattataatgaagatgggggaagggaacacgcagtcatgcccataactgaggattgcaccttttacaaggtgtgcttctgtattatataatttttttaacaggcaggtataaaacttttgtcagccaggcgcggtggctcacgcctgtaatcccagcattatgggaggccgaggcgggcggatcacgaggtcaggagatcgagaccatcctggctaacacagtgagaccccatctctactaaaaatacaaaaaattagccaggcgtgatggtgggcgcctgtagtcccagctactcgggaggctgaggcaggagaatggcgtgaacctgggaggcagaggtggcagtgagctgagattgcgccactgcactgcagcctgagtgaagagtgagactccgtttcaaaaaaaaaaaaaaaaacaacaaaaaaaaaacttttgtcattaaagataaacaagtaaataaagtggacaaagaacagcaactgttgtcatcactggtggggagtgaagtgctgtaggcagcatgggctccagaaggagggtgtcctggagccctgtgggtttgcaagaagatcagttgatggggagctgggatggagcccaagaagcagagaggtgagagcagagtactgtcctggccagctgaggggactcaccaccgtccagggctgctgggagagctgcaacgctgatcacaaatccatgggagatgtctcgacatctgtgttccaggaaagccagaggtcttcttaaggtggttgaatcactctatgccacacagagtctccagaagaccagttcctcactgggagctttctcaaagcttggcgtgtctgccagagctggagcagcagccagagggacgcctctccccctgggctcagcaaaagctcccagacgtcgtctcttccaagttccaccgcacagccagctctttctcttcactgggaggttccgcaggggctgacttgctccttaaggtcccaagactattaagggacacccagtgaggctgggaaaggggctctaagaggcatggacgaagagtcgggggtaaccaagccactggaagctcctggagactcgaggcagagcgaatcttgatgacacaggaatccgtgctgcctcccggtgcagtgtcccagctgggaggagttgaaagac

SEQ ID NO: 14060 - RNA, 260 nt, Homo sapiens
  source 1..260: mol_type = other RNA
gctgggattacaggcatgagccaccgcacccggcctgggtcaagttgcataactctggacacactttggggattaggttattctgaaggactagagtcttcaggccaggcagttttcctaatgctgagggcatctttgtcatcttcttcccattcaaagtaatgatcttcgtatttttaccaccactcaatgcttttattaacaatctctcagtcatgatcttggaaaagaagtagaaaacaaggtaaccattagagttc

SEQ ID NO: 14061 - RNA, 9335 nt, Homo sapiens
  source 1..9335: mol_type = other RNA
gctgggattacaggcatgagccaccgcacccggcctggttttttttttttgttttttttttttaatgaatattacgcttttcattgtagaaactctggaaaacacgtttgtattaatttaggttttgctacataataaaccaccccaaacttttttcttttttcctgagacagggtcttggtgtattgcctaggctggggtgcagtggcatgaatgtggctcattacagcttcgacttcctgggctcaagcaatcctcctgcctcagtttcctgagtggctgggaccacaggcacacaccatcatgcctggctattttctttaatttttttttgtagagatggggtctcatcatgttgcctaggctggtctcaaactcctgggctcaagtgatcctcctgccttggcttcccaaagtactgggaatataggtgtgagccattagacccagccagtttttttattttttatttttattattttacactgtgttgagataaccacccccaaaattagtggcttaagacagcatacattcaggtcacaattctgctggcagtaatttaaatgggctcagagggcagttcttccagtctgggccaacctcagctgttgtcattggggctcactcaaacgtatgaggcatcagctgggatgtcaggatcagctcctccatgtggcctcccatcctacagcagactagcttgggcttgttctcttggagaaggagaagaggagccaagagagcaagcagaaatccacaatgctcttgggcctgtgtctggagctggtaaaacagtacttcccctctgcctcagtcagctcaggctgctgtcacagaacatcatagactggatagcataaacaacacacacttatatctcaccattctggtggctgggaaagtcaagataaaggtgctggcagattcagttgctatgaggacccttatcctggcttgcagaaggctgcttgctgtcttctcattgagtcctcacatgggggtagatggggtgtgtgtgagagagagccagagagacagtgagcacatgctctggtgtttcttcttttccttataaggacactaatcccatgatgggggccctacccacataacctcatttaaacgtaatcatcttccaaaggcccccatctccaaatactaccacactgggagttaggccttcaacataggaattttggagggacacagacactccccaacaccctctattgtacaaagcaagtcacaaggccagcccagattcaaggagtgaagaagtgtaccctacctcttggtgagaagaaatataaaataatattgcattgtgatatgggtggcagcaagtgagggtgagtgggatgaatgtttgcagccatttttgcaaacattttttcataacatacaaaaataaacatctactttaagtcatttctaataccattatcaagagctaattattgttaatatgttggtctatgcacaaataggggcagatatgcacgtacagaggcatagttttgtctgtacacatacagaggcagattgcttttaagaatataattttcatttagaatcaaacttatgttctattagtgtattttcccaggtattaaattttccttgaaaacatgtttaccctatgatgcaaaggaaatcaacataaattactatgttccaggcattgtgctaagcactttcactcagttatcttaactaaaaaacaagtttcttgttaatttgcagggttaatttgcatcaaaacaaggaattcatttgttgctacaaagaaaaagcaatgaaaggactttgtgaaaaggttcagagaaaatgataatggttaagacatatcagcaatacccatttttctcttgaaacctgacttgtgaactataacagaaaatacagaagataaatccttgtacctattgcccaccaatccagtctttccattttataggtgaagtcatgtcattatttatgtatttgtttgatttggctgtatttcaggatcatgttgaacatcagttcttattgtatgggtaacataaataagaagcagaaaatgtagagggcaaaggccaaagtttgatcctgggcttgggactgattagttgttgactatgaaaaaaaaatcacttaatttttttgagttcaattttatcatctgtaattacaaaagcttcaatcttcttaaaattggtgtgaagattgactacagcattttatatctgcactgtctgatgtagtagccactggctataagtggctattgagcatttgaaatgtggctagtccaattgagatgtgctgtaagtataaaatacacagtagattttgaacacttaggtggaaaaatatataaaatatcttattgattacatgttgaaatggcaatatattgtacccattgagttaaataaagtgttattaaaattaattcacttgtttattttttaaattcacttgtaaaaatttattttggctgctggaaattaaaatattacacatatggctcacattatatttctgctggacaatgttttgcttaaaaaatgttctctgtacaatatagagtacagcataaatgttagttatagccagaaaaaaagtataggaggtttagttgaatatgtaaggattctaagtggtagcatgatgcttattatttttgctacatttataatgtaagcttttatttaggcatctgaagtttttctttttatgtgttatagagaagtagggatggaagtgctaatccaattatgtgaggaaatcataataacttcagtgtattgagctacagtgatgcaggcattgtgttaagtactgtattaggcaggattcctttgattacaagtgacagagatgcaatctgaattaactaaattgaaaaagggggatcttgtaattgtatgaagcatgggagtgcatctgggtctcctgaatttctagaatataaacactgtttttcctatatacctatcttcctctctcaaatttacttctccctcctcagcagcattgttctctcagatcacttgtctccatatgtcagaaagaatggctccttcaacctctgtgtgtcatctttgctctagggaaggatagactcagacttgctctttctggttttaaatggaaaagtcctgtgaaaaagccatggttgacctagcttggttataggtacctatccctgggctatggcagctctaacccaaccacagaagagaatttcccagaaaaagggaccattcttcttggttgataaaagaataaatgtacactatagctactctagctaatttaatatgtacagccaatcagtagggtagtacctcaatgaacaaatgagaaactgagactcagaaaagttatgtatttcattcaagttcaaatatccaggctggaagtctgggtctgtccatctccaaagcccatgttcttaactaccacactgagaaagttctagtaaatggggtttgtgtcgacttaagttttactgaattatttaataggtctttgctatttttttcctcctatcattgcttcccattgaaagttaagatagattgaggacaagggaactggccccatggtaatactcagtaaatccttatggaattgaaaaccaacaccactatgctctccaatcttgtgaccaaggctataaaggcgttagaaaagcactgctatcattatctttgtaccatgagcttaagacatagttaccactacttggacatttcctttttgtaatttgcagtcttctgccttcttttgaaaacttcttatttttcaccaacacatggttccctatagtctataccacatgggcatagagatttcagaggcaaagatgaaagagtcatactctgttattcataaataaaatatagccaaagggaattttaaaaaatgatgatctgtaagtctttcagaaaaatggtctggagtttgtcagtctcctactcggatcaaaaataaagtcaaagttttcaactaaaataattgcaataggctacaaatctgtttgtctactttaatacagtagaaatggaaagtagaagtaagtgacaactttattggctgaattcatattaagcagtgtgatggaatgctgagaactctgacccggactggtcagaaaaccagtctcctatatgtagctctgtgaccttaatcagtaataagtacaaaggctaactaaccttcattgggtgctaaacagcgtagaacatcttttcataggttgttgactgactctgcccagtggcagtagttattcattcattcgacacatctttttttttttttttttttgagacggagtctagctctgtcactcaggctggagtgcagtggcgcgatcttagctcactgcaacatccaccttctgggttcaagcaattctctgcctcagcctcctgagtagctgggattaaaggcgcacgccaccacgcctggctaattatttgtatttttattagagacggggtttcaccatgttggccaggctggtcttgaactcctgacctcgtgatccacctgcctcggcctccaaaagtgctgggattacaggagtgagccaccacgcccagcctcattcagcacatctttatcaggcatctaccctgtgtcaggcatggagttaggtaccaaatatggttctgctatcatggagcttacagtctggtgtgggaagtcatacatgtaaacaggcaatttcagtgtagcatgttgtaagtgctatgttagaagaagtagactgttctatgggacctcataaaatgatatcaaacgtggttttgagaaattggatggtttcctgggacatgctgtccatttagggatctgaagggcaggctgggattggccaggtgggggatcacaacaaagctctttgtctggacttagaaagaggttgggaagggggaagtggtgaaggctgagggctgagtcttgagggaaattagctggtcctagaatgcagagtccattatgctgactacctttgactgagggtgataggaaacccttgaatagttttaagcaactgagtcacataattagatctgcattttagaaagctgagatgtgaatcaattttttcatttttctgtcttgattttcttatctttaaattgaaagggatagtctaccctttataactctgtccagctttagtagtccatacatttctcctattttggcaaaacttaatgaaactgcctttgcaaaaattataacagtgagaaaattatgacagtgacagatctgacttaatgactccattttgctattctaaccttcaagctgcccttgttcattgttgggcgcaggctgaactaagtttgggaggaacttagtttaaccttgaaacaaagatgataacagcccttcttgcctgaaaccagactgcccatgtaggactaataaattagctgcaagattggaaatgtaggtttaggagtcctgtagccggaggctgcaagttctgaacctcccccattgctccttggggtaacatcattattgtgaaacctaagattggtctgagatgtttttcagaccttgcattctgaggcaccagctggcgccacccagactggtaatctggcacaaccagttctgcagtgcctcccaggaacagaagacagcaagaagaacccactttaaccccctatgattccatctgtgacccaatcaatcagcactccccactccctggctccccctacgtgccaaatcatcctttaaaaaaaaccctagtgtctgaattttccagggagactgaatcgagtaataaaactctgatctcccattcagttggctctgtgtgaattacactctttctctattacaattcccctgtcttgataaattggctcttatctgggcagtgggcaaggtgaactagttggatgattacgttacttccatgctgattttgagatctgttgggcagcaaggcctaagattacaactagtacttgaaaatgaggcaagttttgtgggtctagggtgggtgaaggtgggaggtgaggtgaggacaagaagctgaatgaatgatgtgttgtttttactgggaaaaaaggaaatgggaaggtatgcagtttcctttgacagtctcctgaagagaaactggttaggaaatagctttggcctctcagcaagcaggtggaatggtactttgccacaattctagtacagatgaaatctgatagttacttcccccaaattatgaagtctggaatttgcttaacggtagtagttaggggtctatacatatgaaaaaagactgaccatgactttttttttttaaccgttcaaagtgtttgttaattatttattaagataaacaatttcttagcccacatattcatgtttcacagatagttcaggaacacaggtacagtgacaaacttctatgtaattcaacccaaagaaatactttatgttccaaaatcactttgtactctgagagatattagccttcctcatctcaaattctttaattcaattataatttctgtagaaatctgcatatgccttctttcttggtcaggccacagcaaacttacagagagctgcaaccccagggttataaggaatgctccaacaatatgaaatgacagatgcttggccagaaggccacacatcccaggttacaccaaggcactgagagccatggtagttattgtccttgacagggatgtcagcatcaacactaatgtctttcccggatgatggagaaatggaccaacttgataagtattgatgctgagtgatacatacaaagaagtccattatatgattttccctacttttgaatatgtttgaaaatttccctaatagaaagtaaaaagatagaataataaaataaaaatacccccacttattacctaagttttcttttagcacaaatggaaaataagtcagactctctcatttggccatattgaagctaatagtctcagaaccactgtgtcataacactgacattttgcttaaagctctgtatcacctttaatggcttaaaatattctagactgtattgagatcatgcaagtagatcaaagaaagagaattacacgcaaaggaagggatagctgtactagggagttcactggtaacagagtcaggggtccacagctctgggctgggtctgtcctgaaaggcagtctctggatagcaggatgagatggagtgatcactggctttggagtcagacacaatagactgagctatgttgaaggacaatgacaaataacacaatagatagcattcattgaaccctcactatatgccaggccttatgctaagctctttatgtactttatgttatgcaattttaataactaccctgtttttattagtattttatggatgagaaaacacaggtttagaggttatcaaatttgtccatgaccacatgaacttgtaattcccagtaaatatttttgtaaataaatatctgaaagtgtccaggcacggtggctcatgcctgcaatcccagcactttgggaggccgaggtaggcggatcacctgaggtcaagagtttgagaccagcctggccaacatgctgaaaccccgtctctactaaaaacacaaaagaattagctgggcatggtggtgtgtgcttgtaatcccagccacttgggaggctgaggcaggagaattgcttgaacccgggaggtgagtcaagattgcgccactgcactccagcctgggcaacaagagtgtgaaaactccatctcaaaaaaaaaaaaaaaaaaaagaaaaaaagtctgaaatccagtggttaatggtggtaggttgtaccccagttagtttggatgcacataacagaaaaaagcaaaataacagtggcaaaataataactaagtagtttgtttttctctcacctctaagtaatctagaggtaatcagtctagggttgctagggctctctggagctcggggttcttctattttactgtttcattgtgaatgtcttccaccctcaaggttaactcatggtccaagtacctgctggagctccatattccaactagaagaaagggagaaggattggaaggacataccacctaccctcctttttaaggatccataccagaaattgcacatattatttttgcttataattacaatggctacaacttagtcctatgtatgcatctagtagattacagaaaacttgcatgtggcaggtccaagacatgaaagagactgaaaaatatttatactatgtggccacatgcccagctaaagggcacagaagcatagaagatggagagcaacattgaggatcactagcaatcactgcttagcccacactcagctgcattccagagttttatctctttgggtatggtaatccttctcacgaaacctttcacattcgaatggataaatacatgaaaaacccatgcacttagtttagtgttcagaaaatgctagttccttccctttaattagatgttgtcaagtgagcagcagtgatttggtgctctggagactcagcaccctaagaatttgttccacctgtgtctggggtggtgactgccttctgcatcaccatcttagaggatttgccccaagttctacatcctctatggcccagcaccctgttaggtacaatggggttgcaaaatgaagcatccagattttaaggatcttgaacataaaatcacacataatgggctcagggccaaacatgggactatccaggatttaggaaaactttcacttcagtgttggtttgcagctgactttgggaaactatttaccacataaaaatttccagtgttttcttcaagactgagagaagtcgatcacagaaccagcccacttgagaagctgaagttttcctacttgtaaaatgacagatgaaaaggactgatgcttccatgagttgctcttgaaatggtaatgtaggtgtatcttgatctcttagcccaccccaaaagtgatgtggcatctgctgtgacaggatagcatttggaatgaggtgtgtatgaaggggatggggtggaatagagcctggttcctcagtattcctcagtgtcactaatcttcatcaagttaataaagcaccagagtttatccaggttttgttcagatccagaacttatacaatgtcggagtcttcttttaagaatacacgatgacagatacaaaattaggtacacagcttaattaacttcatgataaattctcttctgattatgagttactgctttctccctttccttccctccccgcgggccagcggctttggcgctgccctgctgcgcggcggggcgacgcggcgacacctataggattgctt

SEQ ID NO: 14062 - RNA, 9436 nt, Homo sapiens
  source 1..9436: mol_type = other RNA
gctgggattacaggcatgagccaccgcacccggcctggttttttttttttgttttttttttttaatgaatattacgcttttcattgtagaaactctggaaaacacgtttgtattaatttaggttttgctacataataaaccaccccaaacttttttcttttttcctgagacagggtcttggtgtattgcctaggctggggtgcagtggcatgaatgtggctcattacagcttcgacttcctgggctcaagcaatcctcctgcctcagtttcctgagtggctgggaccacaggcacacaccatcatgcctggctattttctttaatttttttttgtagagatggggtctcatcatgttgcctaggctggtctcaaactcctgggctcaagtgatcctcctgccttggcttcccaaagtactgggaatataggtgtgagccattagacccagccagtttttttattttttatttttattattttacactgtgttgagataaccacccccaaaattagtggcttaagacagcatacattcaggtcacaattctgctggcagtaatttaaatgggctcagagggcagttcttccagtctgggccaacctcagctgttgtcattggggctcactcaaacgtatgaggcatcagctgggatgtcaggatcagctcctccatgtggcctcccatcctacagcagactagcttgggcttgttctcttggagaaggagaagaggagccaagagagcaagcagaaatccacaatgctcttgggcctgtgtctggagctggtaaaacagtacttcccctctgcctcagtcagctcaggctgctgtcacagaacatcatagactggatagcataaacaacacacacttatatctcaccattctggtggctgggaaagtcaagataaaggtgctggcagattcagttgctatgaggacccttatcctggcttgcagaaggctgcttgctgtcttctcattgagtcctcacatgggggtagatggggtgtgtgtgagagagagccagagagacagtgagcacatgctctggtgtttcttcttttccttataaggacactaatcccatgatgggggccctacccacataacctcatttaaacgtaatcatcttccaaaggcccccatctccaaatactaccacactgggagttaggccttcaacataggaattttggagggacacagacactccccaacaccctctattgtacaaagcaagtcacaaggccagcccagattcaaggagtgaagaagtgtaccctacctcttggtgagaagaaatataaaataatattgcattgtgatatgggtggcagcaagtgagggtgagtgggatgaatgtttgcagccatttttgcaaacattttttcataacatacaaaaataaacatctactttaagtcatttctaataccattatcaagagctaattattgttaatatgttggtctatgcacaaataggggcagatatgcacgtacagaggcatagttttgtctgtacacatacagaggcagattgcttttaagaatataattttcatttagaatcaaacttatgttctattagtgtattttcccaggtattaaattttccttgaaaacatgtttaccctatgatgcaaaggaaatcaacataaattactatgttccaggcattgtgctaagcactttcactcagttatcttaactaaaaaacaagtttcttgttaatttgcagggttaatttgcatcaaaacaaggaattcatttgttgctacaaagaaaaagcaatgaaaggactttgtgaaaaggttcagagaaaatgataatggttaagacatatcagcaatacccatttttctcttgaaacctgacttgtgaactataacagaaaatacagaagataaatccttgtacctattgcccaccaatccagtctttccattttataggtgaagtcatgtcattatttatgtatttgtttgatttggctgtatttcaggatcatgttgaacatcagttcttattgtatgggtaacataaataagaagcagaaaatgtagagggcaaaggccaaagtttgatcctgggcttgggactgattagttgttgactatgaaaaaaaaatcacttaatttttttgagttcaattttatcatctgtaattacaaaagcttcaatcttcttaaaattggtgtgaagattgactacagcattttatatctgcactgtctgatgtagtagccactggctataagtggctattgagcatttgaaatgtggctagtccaattgagatgtgctgtaagtataaaatacacagtagattttgaacacttaggtggaaaaatatataaaatatcttattgattacatgttgaaatggcaatatattgtacccattgagttaaataaagtgttattaaaattaattcacttgtttattttttaaattcacttgtaaaaatttattttggctgctggaaattaaaatattacacatatggctcacattatatttctgctggacaatgttttgcttaaaaaatgttctctgtacaatatagagtacagcataaatgttagttatagccagaaaaaaagtataggaggtttagttgaatatgtaaggattctaagtggtagcatgatgcttattatttttgctacatttataatgtaagcttttatttaggcatctgaagtttttctttttatgtgttatagagaagtagggatggaagtgctaatccaattatgtgaggaaatcataataacttcagtgtattgagctacagtgatgcaggcattgtgttaagtactgtattaggcaggattcctttgattacaagtgacagagatgcaatctgaattaactaaattgaaaaagggggatcttgtaattgtatgaagcatgggagtgcatctgggtctcctgaatttctagaatataaacactgtttttcctatatacctatcttcctctctcaaatttacttctccctcctcagcagcattgttctctcagatcacttgtctccatatgtcagaaagaatggctccttcaacctctgtgtgtcatctttgctctagggaaggatagactcagacttgctctttctggttttaaatggaaaagtcctgtgaaaaagccatggttgacctagcttggttataggtacctatccctgggctatggcagctctaacccaaccacagaagagaatttcccagaaaaagggaccattcttcttggttgataaaagaataaatgtacactatagctactctagctaatttaatatgtacagccaatcagtagggtagtacctcaatgaacaaatgagaaactgagactcagaaaagttatgtatttcattcaagttcaaatatccaggctggaagtctgggtctgtccatctccaaagcccatgttcttaactaccacactgagaaagttctagtaaatggggtttgtgtcgacttaagttttactgaattatttaataggtctttgctatttttttcctcctatcattgcttcccattgaaagttaagatagattgaggacaagggaactggccccatggtaatactcagtaaatccttatggaattgaaaaccaacaccactatgctctccaatcttgtgaccaaggctataaaggcgttagaaaagcactgctatcattatctttgtaccatgagcttaagacatagttaccactacttggacatttcctttttgtaatttgcagtcttctgccttcttttgaaaacttcttatttttcaccaacacatggttccctatagtctataccacatgggcatagagatttcagaggcaaagatgaaagagtcatactctgttattcataaataaaatatagccaaagggaattttaaaaaatgatgatctgtaagtctttcagaaaaatggtctggagtttgtcagtctcctactcggatcaaaaataaagtcaaagttttcaactaaaataattgcaataggctacaaatctgtttgtctactttaatacagtagaaatggaaagtagaagtaagtgacaactttattggctgaattcatattaagcagtgtgatggaatgctgagaactctgacccggactggtcagaaaaccagtctcctatatgtagctctgtgaccttaatcagtaataagtacaaaggctaactaaccttcattgggtgctaaacagcgtagaacatcttttcataggttgttgactgactctgcccagtggcagtagttattcattcattcgacacatctttttttttttttttttttgagacggagtctagctctgtcactcaggctggagtgcagtggcgcgatcttagctcactgcaacatccaccttctgggttcaagcaattctctgcctcagcctcctgagtagctgggattaaaggcgcacgccaccacgcctggctaattatttgtatttttattagagacggggtttcaccatgttggccaggctggtcttgaactcctgacctcgtgatccacctgcctcggcctccaaaagtgctgggattacaggagtgagccaccacgcccagcctcattcagcacatctttatcaggcatctaccctgtgtcaggcatggagttaggtaccaaatatggttctgctatcatggagcttacagtctggtgtgggaagtcatacatgtaaacaggcaatttcagtgtagcatgttgtaagtgctatgttagaagaagtagactgttctatgggacctcataaaatgatatcaaacgtggttttgagaaattggatggtttcctgggacatgctgtccatttagggatctgaagggcaggctgggattggccaggtgggggatcacaacaaagctctttgtctggacttagaaagaggttgggaagggggaagtggtgaaggctgagggctgagtcttgagggaaattagctggtcctagaatgcagagtccattatgctgactacctttgactgagggtgataggaaacccttgaatagttttaagcaactgagtcacataattagatctgcattttagaaagctgagatgtgaatcaattttttcatttttctgtcttgattttcttatctttaaattgaaagggatagtctaccctttataactctgtccagctttagtagtccatacatttctcctattttggcaaaacttaatgaaactgcctttgcaaaaattataacagtgagaaaattatgacagtgacagatctgacttaatgactccattttgctattctaaccttcaagctgcccttgttcattgttgggcgcaggctgaactaagtttgggaggaacttagtttaaccttgaaacaaagatgataacagcccttcttgcctgaaaccagactgcccatgtaggactaataaattagctgcaagattggaaatgtaggtttaggagtcctgtagccggaggctgcaagttctgaacctcccccattgctccttggggtaacatcattattgtgaaacctaagattggtctgagatgtttttcagaccttgcattctgaggcaccagctggcgccacccagactggtaatctggcacaaccagttctgcagtgcctcccaggaacagaagacagcaagaagaacccactttaaccccctatgattccatctgtgacccaatcaatcagcactccccactccctggctccccctacgtgccaaatcatcctttaaaaaaaaccctagtgtctgaattttccagggagactgaatcgagtaataaaactctgatctcccattcagttggctctgtgtgaattacactctttctctattacaattcccctgtcttgataaattggctcttatctgggcagtgggcaaggtgaactagttggatgattacgttacttccatgctgattttgagatctgttgggcagcaaggcctaagattacaactagtacttgaaaatgaggcaagttttgtgggtctagggtgggtgaaggtgggaggtgaggtgaggacaagaagctgaatgaatgatgtgttgtttttactgggaaaaaaggaaatgggaaggtatgcagtttcctttgacagtctcctgaagagaaactggttaggaaatagctttggcctctcagcaagcaggtggaatggtactttgccacaattctagtacagatgaaatctgatagttacttcccccaaattatgaagtctggaatttgcttaacggtagtagttaggggtctatacatatgaaaaaagactgaccatgactttttttttttaaccgttcaaagtgtttgttaattatttattaagataaacaatttcttagcccacatattcatgtttcacagatagttcaggaacacaggtacagtgacaaacttctatgtaattcaacccaaagaaatactttatgttccaaaatcactttgtactctgagagatattagccttcctcatctcaaattctttaattcaattataatttctgtagaaatctgcatatgccttctttcttggtcaggccacagcaaacttacagagagctgcaaccccagggttataaggaatgctccaacaatatgaaatgacagatgcttggccagaaggccacacatcccaggttacaccaaggcactgagagccatggtagttattgtccttgacagggatgtcagcatcaacactaatgtctttcccggatgatggagaaatggaccaacttgataagtattgatgctgagtgatacatacaaagaagtccattatatgattttccctacttttgaatatgtttgaaaatttccctaatagaaagtaaaaagatagaataataaaataaaaatacccccacttattacctaagttttcttttagcacaaatggaaaataagtcagactctctcatttggccatattgaagctaatagtctcagaaccactgtgtcataacactgacattttgcttaaagctctgtatcacctttaatggcttaaaatattctagactgtattgagatcatgcaagtagatcaaagaaagagaattacacgcaaaggaagggatagctgtactagggagttcactggtaacagagtcaggggtccacagctctgggctgggtctgtcctgaaaggcagtctctggatagcaggatgagatggagtgatcactggctttggagtcagacacaatagactgagctatgttgaaggacaatgacaaataacacaatagatagcattcattgaaccctcactatatgccaggccttatgctaagctctttatgtactttatgttatgcaattttaataactaccctgtttttattagtattttatggatgagaaaacacaggtttagaggttatcaaatttgtccatgaccacatgaacttgtaattcccagtaaatatttttgtaaataaatatctgaaagtgtccaggcacggtggctcatgcctgcaatcccagcactttgggaggccgaggtaggcggatcacctgaggtcaagagtttgagaccagcctggccaacatgctgaaaccccgtctctactaaaaacacaaaagaattagctgggcatggtggtgtgtgcttgtaatcccagccacttgggaggctgaggcaggagaattgcttgaacccgggaggtgagtcaagattgcgccactgcactccagcctgggcaacaagagtgtgaaaactccatctcaaaaaaaaaaaaaaaaaaaagaaaaaaagtctgaaatccagtggttaatggtggtaggttgtaccccagttagtttggatgcacataacagaaaaaagcaaaataacagtggcaaaataataactaagtagtttgtttttctctcacctctaagtaatctagaggtaatcagtctagggttgctagggctctctggagctcggggttcttctattttactgtttcattgtgaatgtcttccaccctcaaggttaactcatggtccaagtacctgctggagctccatattccaactagaagaaagggagaaggattggaaggacataccacctaccctcctttttaaggatccataccagaaattgcacatattatttttgcttataattacaatggctacaacttagtcctatgtatgcatctagtagattacagaaaacttgcatgtggcaggtccaagacatgaaagagactgaaaaatatttatactatgtggccacatgcccagctaaagggcacagaagcatagaagatggagagcaacattgaggatcactagcaatcactgcttagcccacactcagctgcattccagagttttatctctttgggtatggtaatccttctcacgaaacctttcacattcgaatggataaatacatgaaaaacccatgcacttagtttagtgttcagaaaatgctagttccttccctttaattagatgttgtcaagtgagcagcagtgatttggtgctctggagactcagcaccctaagaatttgttccacctgtgtctggggtggtgactgccttctgcatcaccatcttagaggatttgccccaagttctacatcctctatggcccagcaccctgttaggtacaatggggttgcaaaatgaagcatccagattttaaggatcttgaacataaaatcacacataatgggctcagggccaaacatgggactatccaggatttaggaaaactttcacttcagtgttggtttgcagctgactttgggaaactatttaccacataaaaatttccagtgttttcttcaagactgagagaagtcgatcacagaaccagcccacttgagaagctgaagttttcctacttgtaaaatgacagatgaaaaggactgatgcttccatgagttgctcttgaaatggtaatgtaggtgtatcttgatctcttagcccaccccaaaagtgatgtggcatctgctgtgacaggatagcatttggaatgaggtgtgtatgaaggggatggggtggaatagagcctggttcctcagtattcctcagtgtcactaatcttcatcaagttaataaagcaccagagtttatccaggttttgttcagatccagaacttatacaatgtcggagtcttcttttaagaatacacgatgacagatacaaaattaggtacacagcttaattaacttcatgataaattctcttctgattatgagttactgctttctttggccagaattgtgaaagaaaaataaggcgtgaggctagaggatggggaaaaaaaatccttgtctatcttgcttcccaagcaggccttcaagctagctaactgaaacagtcttttctccaggtcctaaggtaaatggtggcggatctgaaaatgcgtcggacttaaccttgcccttctccccagttt

SEQ ID NO: 14063 - RNA, 5431 nt, Homo sapiens
  source 1..5431: mol_type = other RNA
gctgggattacaggcatgagccaccgcacccggcctgtttattttgtttgtttgtttaactccccctgcacctccgccaaaaaaaaaaaaataaaagaaaaagaaaaactaacctgtaactctgaagtgtctggtagccaggtgcggtggctcgcacctgtaatcccagcactttgggaggtcgaggtgggcagatcatttgaggtcaggagtttgaaaccagcctgaccaacatggtgaaaccctgtctctactaaaaatacaattacctgggcatggtggcgcacacctgtaatcccagctacttgggaggctgaggcagaattgcttgagttcgggaggcagatgttgcaatgagcagagattgcactccagcctaggtgacagagcgatactctggctcaaaaaaaataaaataataaagtctcttgcctttggagtcgggcatgaaatcttaatccgtgagttttctacctgggccatggtgggccactgaccaccttcggcctggatgaaggctggcccccagagggttgccaagctttgccagtgctccctggcctgcgtggggcctggctgagggcgagggcaacaggaatgcattgtgtctggggctgagcaggacttgcggtgcctgggccctttgagcctggtgactcctgagtgtgactcctgagtctgaccccatcacccgtgtgggctgacaccagcaccttccacgctgtgcttctgtgtttgccgccggtctccaggagtggccgcttctccatcaaataatactccagtcttcacgcccatggcttcccccagaccccagcccagcccgagaacaaacgctccattttccctcccttacagctgcggtggttgccaccacatggaaggcccagaggaagggaggtctggagtggcctggagctgtggcctccccaggctacggccagacccaccaggaggaagccccttgcaggctctaaggttaacgccgccaaaccaagtcctgatcctgagaggctggctcaggatgaggatgggcggtggtgtcatgcacaggcacctgaggtccctggctgctgtggcacggagaggcccccacggaaggactccgcaggtgctggagctcgctccctgcatggacagctgcagcctgggcagggataggggagcaaagctgcaggcccggctcatcatggaaattcagaccggtgagccatggaaggacatcgccaagtccatgtagggtgagctggggacagcatggggagtgggaggggggacagtggggagaggggagagcggggtgagctgggtacagcatggggagggggacagtggggaggggggagagcggggggagcctggggacagcatggggagtggtgggggtgggggaaggtggagggagggcagtgcatggaggacagtggaagagggaggcagtggtgacagtggagagggaagacagtggggaggtagaagggaggagggtaggacagtccagcccccattggcaggggcagctggggagagcaggccccgcctttgtgtgccccagggcctgggcctgcctggttaagagtctgcacactcctagagctggagcttctcaatgtcgctcttggaaggtgaccccacactccgctggggataatgcagggggcccaggggtcctccctgggaaaagtgtgctgtgccccgccatagggttcgtggcagaagcccctcccctgagctcaggcctcacctccggccactgaagacaaggagatgcagagaggaggcctctggagtcttgccccttacccctgcacccctgcagcacaggcagggtgtggtggccgtcttggaggcacccgggcctggacagctattccaaagccatagctgccctccccagggtgggtcgcttggtcttaggagcgtccaagctgcagagcccagtagacagaacctggatccagcgcctcactttacaggaggggaaactgaggcacaagcatgtgctacctggctcgggggccagcaggcagccttttcccttctgtcacctgccctagggatggaccgccccatctgccagccttgactggagcctccctggtggatgtttaccgcacacctactacgtgcagggtggtgcagctggcgagagtcccctctcctgttccacagaccggcaaggttcccctgagccctggggcaggcaggacctttggctggaggtgggtgtgcagggcagggtctctgaggggagacctcagactgtggacttgcgggtggacgcttctctctgtcggggcctcccgtgtccagaagatgttgaacagcatctgaggcttccacccgctgaagccgaggaacagcccccagctgtgacaacccaaaatgcctccagacctggccccatgtcctccagggggacggaacagcctggtgtagggcagggtcccctgagcaggagtggcacctgttcctgctcataccacagacagctgagctggctgtgcccaagactccctgcacccaccaaagccactggatacaggcacgatttgcatcttactctcttaagtcaggtttctggagatggctgtcccaacactggaatccagcctgtctacagcaagggagaaagaggaagctgatgttgggctgagaggggcaggcgttacagggtaggtctcacaaatgccgacgtgacaggcagggcttctgagggggcttcagggaccagcagggaggcgagactcaggcactgacccgcagagagcatggccttggacgcacagtggtgacagcagcctccaagtgtcccccgtgccctcaggcatgagggacagaagcttctggggcccctgcctctttcctgcccatcccctggtgaaggaaaatcgcctctgataggaaaagctggggccagactccctctccctgcattagtgtcgccgtcctgcctgtgaggtccccgggcccagggcacctcccgggacacccgagtggtgatgcacgaccctcagtcctggggcttaggacctctgggtgcccccgcaggtccgtcctggagtcacttcacagtcactgcaaatgggcaccacagcccactttccaacgccccaactttccacacccaagcagctccttgtccctgccaatcaatgcccggtgatgacaactgttcttttataaacaccacacatcttctaatgctttcatgttaaaagcgggagtggatcccacattcacctaaaggctcaggtagggactttttttgcagaaaaccaatttcttgtaacaagtactggaacctcattgtagccttgagtcctcactcctccttttgttctaagtctgggtctgagaagtgcaggcctcacacagctgtcagttccaagtgaccagggctgtaacaggtcctggctgaccctgggaatgtcaggggattctgggaagtaagaaggaggggcatttgcccatagccccggggcagacaatgtgtcccgagggccaggccaggctgtctactccatctccctggggcgagtgcacctcgggtcacctggcagcatcctttccagcccttctggagacagtcagcagctgattcattccgggaaccagcatggcaggtgccggggctggtcagggcccagggctgtacccctcagcactggaccaccccgtctcctgcccccttgggactgttgggctccgaggagcctggcgctggggtcggaggtcttcatcaggaccctggggaccctcagggttgagtggggtggggctgctgagggtggtgggggccgggggagccacctctcactttggggatcattgctgaggtgagaagggggactgtggccaccaggtgataccctctccatgcacctaactgctgctcaggactctggggaccgtgttgccaggcctgcgcctgctggacatgggcgtctccagccctgctgggctgtgtctttctcgctgcagagccaagagccccggcagcccctgtagccaaacacggccctggcacagcctttcttctggcaaactccacccgtgcgtcttccaaaggtggctcaacttttcaccggaacagccgagggacattgttcctcccagggaatgtggcagaggacactgaagcccagtggggacttccgggggctcctcggtgtggacggctaactacacttgtgggcacacacatgagtgggtcctgtggcttccgggcgggaggcaggttgggagcgttcagggcagaagagctcctgtgaccgtgtcccctgcaaacagcctcgcgtgaccccagcagcacagaggccgtcctggaagagcggacgcccagtcttctttttaaaccaaacacccttcggtctcaggatcccgcatcccacgggaagacccacagtgggtctggggtactgggaagagcctggtgctgaatcccgcacgctccgggtagagacagcccatcaccagtcccttcctgtgggtgactggcagtgacagcggggagcccactcacttggggacatttgcctttggtgtggatgacgcttttgaaagggcctcattccaggatcacagccaacgccagcaggttctccctgggatccagcagtggtccttctgggggctgccccaagtgctcccctgcagtctgggagtccatgctcaagctgccacctggcctctcacggtggcgtctcacggaagccctgtccacgctctgggcggtgagctccggtcaaacgtggccagtgagctctgtctccggactcacagcccaggcacctgcatagctgtgttggaggcatcggtccctgcacacccagcctatggccaccgccacgaccacaagcaggcacaggacagccaggatgctccacgtggccgcgtttttctcgccggtactgactggattctctgtgatcttgtctctctctccgatgtcatttcctgtctggctgccgacagtcaggttctgctgcagaagcacgttctctatgcagcagccaatgttcacgctgggggtccgtgcgatcctcagcacgctgaccacgtcatacaagccccgcatgttcaagaagacggtgtcattctgcagagcctggtccagcaggctgttgtccgtcttattgatccagtacacgttgggcctggggtagccgtttatggatgtacacgtgaaggtgagctcatcctgggaggggctgtggggggcgctgacgacgggcacgctgaagtttgcagctcgaaggctgctgaagagcaggaagagcagtccaggactgcccagccgcatggtgcgggcggagacctcgggccgcggagacctcggggcgcggagacctcggggcgcggagaacttgggccgcgggagacctcggagaggagcaacctcggggcgcgggagatcggctctaactgc

SEQ ID NO: 14064 - RNA, 5630 nt, Homo sapiens
  source 1..5630: mol_type = other RNA
gctgggattacaggcatgagccaccgcacccggcctgtttattttgtttgtttgtttaactccccctgcacctccgccaaaaaaaaaaaaataaaagaaaaagaaaaactaacctgtaactctgaagtgtctggtagccaggtgcggtggctcgcacctgtaatcccagcactttgggaggtcgaggtgggcagatcatttgaggtcaggagtttgaaaccagcctgaccaacatggtgaaaccctgtctctactaaaaatacaattacctgggcatggtggcgcacacctgtaatcccagctacttgggaggctgaggcagaattgcttgagttcgggaggcagatgttgcaatgagcagagattgcactccagcctaggtgacagagcgatactctggctcaaaaaaaataaaataataaagtctcttgcctttggagtcgggcatgaaatcttaatccgtgagttttctacctgggccatggtgggccactgaccaccttcggcctggatgaaggctggcccccagagggttgccaagctttgccagtgctccctggcctgcgtggggcctggctgagggcgagggcaacaggaatgcattgtgtctggggctgagcaggacttgcggtgcctgggccctttgagcctggtgactcctgagtgtgactcctgagtctgaccccatcacccgtgtgggctgacaccagcaccttccacgctgtgcttctgtgtttgccgccggtctccaggagtggccgcttctccatcaaataatactccagtcttcacgcccatggcttcccccagaccccagcccagcccgagaacaaacgctccattttccctcccttacagctgcggtggttgccaccacatggaaggcccagaggaagggaggtctggagtggcctggagctgtggcctccccaggctacggccagacccaccaggaggaagccccttgcaggctctaaggttaacgccgccaaaccaagtcctgatcctgagaggctggctcaggatgaggatgggcggtggtgtcatgcacaggcacctgaggtccctggctgctgtggcacggagaggcccccacggaaggactccgcaggtgctggagctcgctccctgcatggacagctgcagcctgggcagggataggggagcaaagctgcaggcccggctcatcatggaaattcagaccggtgagccatggaaggacatcgccaagtccatgtagggtgagctggggacagcatggggagtgggaggggggacagtggggagaggggagagcggggtgagctgggtacagcatggggagggggacagtggggaggggggagagcggggggagcctggggacagcatggggagtggtgggggtgggggaaggtggagggagggcagtgcatggaggacagtggaagagggaggcagtggtgacagtggagagggaagacagtggggaggtagaagggaggagggtaggacagtccagcccccattggcaggggcagctggggagagcaggccccgcctttgtgtgccccagggcctgggcctgcctggttaagagtctgcacactcctagagctggagcttctcaatgtcgctcttggaaggtgaccccacactccgctggggataatgcagggggcccaggggtcctccctgggaaaagtgtgctgtgccccgccatagggttcgtggcagaagcccctcccctgagctcaggcctcacctccggccactgaagacaaggagatgcagagaggaggcctctggagtcttgccccttacccctgcacccctgcagcacaggcagggtgtggtggccgtcttggaggcacccgggcctggacagctattccaaagccatagctgccctccccagggtgggtcgcttggtcttaggagcgtccaagctgcagagcccagtagacagaacctggatccagcgcctcactttacaggaggggaaactgaggcacaagcatgtgctacctggctcgggggccagcaggcagccttttcccttctgtcacctgccctagggatggaccgccccatctgccagccttgactggagcctccctggtggatgtttaccgcacacctactacgtgcagggtggtgcagctggcgagagtcccctctcctgttccacagaccggcaaggttcccctgagccctggggcaggcaggacctttggctggaggtgggtgtgcagggcagggtctctgaggggagacctcagactgtggacttgcgggtggacgcttctctctgtcggggcctcccgtgtccagaagatgttgaacagcatctgaggcttccacccgctgaagccgaggaacagcccccagctgtgacaacccaaaatgcctccagacctggccccatgtcctccagggggacggaacagcctggtgtagggcagggtcccctgagcaggagtggcacctgttcctgctcataccacagacagctgagctggctgtgcccaagactccctgcacccaccaaagccactggatacaggcacgatttgcatcttactctcttaagtcaggtttctggagatggctgtcccaacactggaatccagcctgtctacagcaagggagaaagaggaagctgatgttgggctgagaggggcaggcgttacagggtaggtctcacaaatgccgacgtgacaggcagggcttctgagggggcttcagggaccagcagggaggcgagactcaggcactgacccgcagagagcatggccttggacgcacagtggtgacagcagcctccaagtgtcccccgtgccctcaggcatgagggacagaagcttctggggcccctgcctctttcctgcccatcccctggtgaaggaaaatcgcctctgataggaaaagctggggccagactccctctccctgcattagtgtcgccgtcctgcctgtgaggtccccgggcccagggcacctcccgggacacccgagtggtgatgcacgaccctcagtcctggggcttaggacctctgggtgcccccgcaggtccgtcctggagtcacttcacagtcactgcaaatgggcaccacagcccactttccaacgccccaactttccacacccaagcagctccttgtccctgccaatcaatgcccggtgatgacaactgttcttttataaacaccacacatcttctaatgctttcatgttaaaagcgggagtggatcccacattcacctaaaggctcaggtagggactttttttgcagaaaaccaatttcttgtaacaagtactggaacctcattgtagccttgagtcctcactcctccttttgttctaagtctgggtctgagaagtgcaggcctcacacagctgtcagttccaagtgaccagggctgtaacaggtcctggctgaccctgggaatgtcaggggattctgggaagtaagaaggaggggcatttgcccatagccccggggcagacaatgtgtcccgagggccaggccaggctgtctactccatctccctggggcgagtgcacctcgggtcacctggcagcatcctttccagcccttctggagacagtcagcagctgattcattccgggaaccagcatggcaggtgccggggctggtcagggcccagggctgtacccctcagcactggaccaccccgtctcctgcccccttgggactgttgggctccgaggagcctggcgctggggtcggaggtcttcatcaggaccctggggaccctcagggttgagtggggtggggctgctgagggtggtgggggccgggggagccacctctcactttggggatcattgctgaggtgagaagggggactgtggccaccaggtgataccctctccatgcacctaactgctgctcaggactctggggaccgtgttgccaggcctgcgcctgctggacatgggcgtctccagccctgctgggctgtgtctttctcgctgcagagccaagagccccggcagcccctgtagccaaacacggccctggcacagcctttcttctggcaaactccacccgtgcgtcttccaaaggtggctcaacttttcaccggaacagccgagggacattgttcctcccagggaatgtggcagaggacactgaagcccagtggggacttccgggggctcctcggtgtggacggctaactacacttgtgggcacacacatgagtgggtcctgtggcttccgggcgggaggcaggttgggagcgttcagggcagaagagctcctgtgaccgtgtcccctgcaaacagcctcgcgtgaccccagcagcacagaggccgtcctggaagagcggacgcccagtcttctttttaaaccaaacacccttcggtctcaggatcccgcatcccacgggaagacccacagtgggtctggggtactgggaagagcctggtgctgaatcccgcacgctccgggtagagacagcccatcaccagtcccttcctgtgggtgactggcagtgacagcggggagcccactcacttggggacatttgcctttggtgtggatgacgcttttgaaagggcctcattccaggatcacagccaacgccagcaggttctccctgggatccagcagtggtccttctgggggctgccccaagtgctcccctgcagtctgggagtccatgctcaagctgccacctggcctctcacggtggcgtctcacggaagccctgtccacgctctgggcggtgagctccggtcaaacgtggccagtgagctctgtctccggactcacagcccaggcacctgcatagctgtgttggaggcatcggtccctgcacacccagcctatggccaccgccacgaccacaagcaggcacaggacagccaggatgctccacgtggccgcgtttttctcgccggtactgactggattctctgtgatcttgtctctctctccgatgtcatttcctgtctggctgccgacagtcaggttctgctgcagaagcacgttctctatgcagcagccaatgttcacgctgggggtccgtgcgatcctcagcacgctgaccacgtcatacaagccccgcatgttcaagaagacggtgtcattctgcagagcctggtccagcaggctgttgtccgtcttattgatccagtacacgttgggcctggggtagccgtttatggatgtacacgtgaaggtgagctcatcctgggaggggctgtggggggcgctgacgacgggcacgctgaagtttgctgccacatgcagtgtaacctcaacgctcaaaacctcctggaatcccagggattggctcaacaccaggcagtgaaacttctgctcgtcctggggggtgacgttgaacaagcgcagggagaagtcgccccgcagcatgccggccggtgacatcagggctcggttccggtagcggctgtccacgttttccaaggagctgttcagctcgaaggctgctgaagagcaggaagagcagtccaggactgcccagccgcatggtgcgggcggagacctcgggccgcggagacctcggggcgcggagacctcggggcgcggagaacttgggccgcgggagacctcggagaggagcaacctcggggcgcgggagatcggctctaactgc

SEQ ID NO: 14065 - RNA, 5782 nt, Homo sapiens
  source 1..5782: mol_type = other RNA
gctgggattacaggcatgagccaccgcacccggcctgtttattttgtttgtttgtttaactccccctgcacctccgccaaaaaaaaaaaaataaaagaaaaagaaaaactaacctgtaactctgaagtgtctggtagccaggtgcggtggctcgcacctgtaatcccagcactttgggaggtcgaggtgggcagatcatttgaggtcaggagtttgaaaccagcctgaccaacatggtgaaaccctgtctctactaaaaatacaattacctgggcatggtggcgcacacctgtaatcccagctacttgggaggctgaggcagaattgcttgagttcgggaggcagatgttgcaatgagcagagattgcactccagcctaggtgacagagcgatactctggctcaaaaaaaataaaataataaagtctcttgcctttggagtcgggcatgaaatcttaatccgtgagttttctacctgggccatggtgggccactgaccaccttcggcctggatgaaggctggcccccagagggttgccaagctttgccagtgctccctggcctgcgtggggcctggctgagggcgagggcaacaggaatgcattgtgtctggggctgagcaggacttgcggtgcctgggccctttgagcctggtgactcctgagtgtgactcctgagtctgaccccatcacccgtgtgggctgacaccagcaccttccacgctgtgcttctgtgtttgccgccggtctccaggagtggccgcttctccatcaaataatactccagtcttcacgcccatggcttcccccagaccccagcccagcccgagaacaaacgctccattttccctcccttacagctgcggtggttgccaccacatggaaggcccagaggaagggaggtctggagtggcctggagctgtggcctccccaggctacggccagacccaccaggaggaagccccttgcaggctctaaggttaacgccgccaaaccaagtcctgatcctgagaggctggctcaggatgaggatgggcggtggtgtcatgcacaggcacctgaggtccctggctgctgtggcacggagaggcccccacggaaggactccgcaggtgctggagctcgctccctgcatggacagctgcagcctgggcagggataggggagcaaagctgcaggcccggctcatcatggaaattcagaccggtgagccatggaaggacatcgccaagtccatgtagggtgagctggggacagcatggggagtgggaggggggacagtggggagaggggagagcggggtgagctgggtacagcatggggagggggacagtggggaggggggagagcggggggagcctggggacagcatggggagtggtgggggtgggggaaggtggagggagggcagtgcatggaggacagtggaagagggaggcagtggtgacagtggagagggaagacagtggggaggtagaagggaggagggtaggacagtccagcccccattggcaggggcagctggggagagcaggccccgcctttgtgtgccccagggcctgggcctgcctggttaagagtctgcacactcctagagctggagcttctcaatgtcgctcttggaaggtgaccccacactccgctggggataatgcagggggcccaggggtcctccctgggaaaagtgtgctgtgccccgccatagggttcgtggcagaagcccctcccctgagctcaggcctcacctccggccactgaagacaaggagatgcagagaggaggcctctggagtcttgccccttacccctgcacccctgcagcacaggcagggtgtggtggccgtcttggaggcacccgggcctggacagctattccaaagccatagctgccctccccagggtgggtcgcttggtcttaggagcgtccaagctgcagagcccagtagacagaacctggatccagcgcctcactttacaggaggggaaactgaggcacaagcatgtgctacctggctcgggggccagcaggcagccttttcccttctgtcacctgccctagggatggaccgccccatctgccagccttgactggagcctccctggtggatgtttaccgcacacctactacgtgcagggtggtgcagctggcgagagtcccctctcctgttccacagaccggcaaggttcccctgagccctggggcaggcaggacctttggctggaggtgggtgtgcagggcagggtctctgaggggagacctcagactgtggacttgcgggtggacgcttctctctgtcggggcctcccgtgtccagaagatgttgaacagcatctgaggcttccacccgctgaagccgaggaacagcccccagctgtgacaacccaaaatgcctccagacctggccccatgtcctccagggggacggaacagcctggtgtagggcagggtcccctgagcaggagtggcacctgttcctgctcataccacagacagctgagctggctgtgcccaagactccctgcacccaccaaagccactggatacaggcacgatttgcatcttactctcttaagtcaggtttctggagatggctgtcccaacactggaatccagcctgtctacagcaagggagaaagaggaagctgatgttgggctgagaggggcaggcgttacagggtaggtctcacaaatgccgacgtgacaggcagggcttctgagggggcttcagggaccagcagggaggcgagactcaggcactgacccgcagagagcatggccttggacgcacagtggtgacagcagcctccaagtgtcccccgtgccctcaggcatgagggacagaagcttctggggcccctgcctctttcctgcccatcccctggtgaaggaaaatcgcctctgataggaaaagctggggccagactccctctccctgcattagtgtcgccgtcctgcctgtgaggtccccgggcccagggcacctcccgggacacccgagtggtgatgcacgaccctcagtcctggggcttaggacctctgggtgcccccgcaggtccgtcctggagtcacttcacagtcactgcaaatgggcaccacagcccactttccaacgccccaactttccacacccaagcagctccttgtccctgccaatcaatgcccggtgatgacaactgttcttttataaacaccacacatcttctaatgctttcatgttaaaagcgggagtggatcccacattcacctaaaggctcaggtagggactttttttgcagaaaaccaatttcttgtaacaagtactggaacctcattgtagccttgagtcctcactcctccttttgttctaagtctgggtctgagaagtgcaggcctcacacagctgtcagttccaagtgaccagggctgtaacaggtcctggctgaccctgggaatgtcaggggattctgggaagtaagaaggaggggcatttgcccatagccccggggcagacaatgtgtcccgagggccaggccaggctgtctactccatctccctggggcgagtgcacctcgggtcacctggcagcatcctttccagcccttctggagacagtcagcagctgattcattccgggaaccagcatggcaggtgccggggctggtcagggcccagggctgtacccctcagcactggaccaccccgtctcctgcccccttgggactgttgggctccgaggagcctggcgctggggtcggaggtcttcatcaggaccctggggaccctcagggttgagtggggtggggctgctgagggtggtgggggccgggggagccacctctcactttggggatcattgctgaggtgagaagggggactgtggccaccaggtgataccctctccatgcacctaactgctgctcaggactctggggaccgtgttgccaggcctgcgcctgctggacatgggcgtctccagccctgctgggctgtgtctttctcgctgcagagccaagagccccggcagcccctgtagccaaacacggccctggcacagcctttcttctggcaaactccacccgtgcgtcttccaaaggtggctcaacttttcaccggaacagccgagggacattgttcctcccagggaatgtggcagaggacactgaagcccagtggggacttccgggggctcctcggtgtggacggctaactacacttgtgggcacacacatgagtgggtcctgtggcttccgggcgggaggcaggttgggagcgttcagggcagaagagctcctgtgaccgtgtcccctgcaaacagcctcgcgtgaccccagcagcacagaggccgtcctggaagagcggacgcccagtcttctttttaaaccaaacacccttcggtctcaggatcccgcatcccacgggaagacccacagtgggtctggggtactgggaagagcctggtgctgaatcccgcacgctccgggtagagacagcccatcaccagtcccttcctgtgggtgactggcagtgacagcggggagcccactcacttggggacatttgcctttggtgtggatgacgcttttgaaagggcctcattccaggatcacagccaacgccagcaggttctccctgggatccagcagtggtccttctgggggctgccccaagtgctcccctgcagtctgggagtccatgctcaagctgccacctggcctctcacggtggcgtctcacggaagccctgtccacgctctgggcggtgagctccggtcaaacgtggccagtgagctctgtctccggactcacagcccaggcacctgcatagctgtgttggaggcatcggtccctgcacacccagcctatggccaccgccacgaccacaagcaggcacaggacagccaggatgctccacgtggccgcgtttttctcgccggtactgactggattctctgtgatcttgtctctctctccgatgtcatttcctgtctggctgccgacagtcaggttctgctgcagaagcacgttctctatgcagcagccaatgttcacgctgggggtccgtgcgatcctcagcacgctgaccacgtcatacaagccccgcatgttcaagaagacggtgtcattctgcagagcctggtccagcaggctgttgtccgtcttattgatccagtacacgttgggcctggggtagccgtttatggatgtacacgtgaaggtgagctcatcctgggaggggctgtggggggcgctgacgacgggcacgctgaagtttgctgccacatgcagtgtaacctcaacgctcaaaacctcctggaatcccagggattggctcaacaccaggcagtgaaacttctgctcgtcctggggggtgacgttgaacaagcgcagggagaagtcgccccgcagcatgccggccggtgacatcagggctcggttccggtagcggctgtccacgttttccaaggagctgttctgtgggatgtggtaggtcaccacggttttcgactcactggtttgccaatatacgtaaacatcatttaaatcaaaacggcttccttcagggcaagcgcagctgagctccacgtcgctgcctaccatcgctctgacttccttctcctgagtatcagctcgaaggctgctgaagagcaggaagagcagtccaggactgcccagccgcatggtgcgggcggagacctcgggccgcggagacctcggggcgcggagacctcggggcgcggagaacttgggccgcgggagacctcggagaggagcaacctcggggcgcgggagatcggctctaactgc

SEQ ID NO: 14066 - RNA, 6118 nt, Homo sapiens
  source 1..6118: mol_type = other RNA
gctgggattacaggcatgagccaccgcacccggcctgtttattttgtttgtttgtttaactccccctgcacctccgccaaaaaaaaaaaaataaaagaaaaagaaaaactaacctgtaactctgaagtgtctggtagccaggtgcggtggctcgcacctgtaatcccagcactttgggaggtcgaggtgggcagatcatttgaggtcaggagtttgaaaccagcctgaccaacatggtgaaaccctgtctctactaaaaatacaattacctgggcatggtggcgcacacctgtaatcccagctacttgggaggctgaggcagaattgcttgagttcgggaggcagatgttgcaatgagcagagattgcactccagcctaggtgacagagcgatactctggctcaaaaaaaataaaataataaagtctcttgcctttggagtcgggcatgaaatcttaatccgtgagttttctacctgggccatggtgggccactgaccaccttcggcctggatgaaggctggcccccagagggttgccaagctttgccagtgctccctggcctgcgtggggcctggctgagggcgagggcaacaggaatgcattgtgtctggggctgagcaggacttgcggtgcctgggccctttgagcctggtgactcctgagtgtgactcctgagtctgaccccatcacccgtgtgggctgacaccagcaccttccacgctgtgcttctgtgtttgccgccggtctccaggagtggccgcttctccatcaaataatactccagtcttcacgcccatggcttcccccagaccccagcccagcccgagaacaaacgctccattttccctcccttacagctgcggtggttgccaccacatggaaggcccagaggaagggaggtctggagtggcctggagctgtggcctccccaggctacggccagacccaccaggaggaagccccttgcaggctctaaggttaacgccgccaaaccaagtcctgatcctgagaggctggctcaggatgaggatgggcggtggtgtcatgcacaggcacctgaggtccctggctgctgtggcacggagaggcccccacggaaggactccgcaggtgctggagctcgctccctgcatggacagctgcagcctgggcagggataggggagcaaagctgcaggcccggctcatcatggaaattcagaccggtgagccatggaaggacatcgccaagtccatgtagggtgagctggggacagcatggggagtgggaggggggacagtggggagaggggagagcggggtgagctgggtacagcatggggagggggacagtggggaggggggagagcggggggagcctggggacagcatggggagtggtgggggtgggggaaggtggagggagggcagtgcatggaggacagtggaagagggaggcagtggtgacagtggagagggaagacagtggggaggtagaagggaggagggtaggacagtccagcccccattggcaggggcagctggggagagcaggccccgcctttgtgtgccccagggcctgggcctgcctggttaagagtctgcacactcctagagctggagcttctcaatgtcgctcttggaaggtgaccccacactccgctggggataatgcagggggcccaggggtcctccctgggaaaagtgtgctgtgccccgccatagggttcgtggcagaagcccctcccctgagctcaggcctcacctccggccactgaagacaaggagatgcagagaggaggcctctggagtcttgccccttacccctgcacccctgcagcacaggcagggtgtggtggccgtcttggaggcacccgggcctggacagctattccaaagccatagctgccctccccagggtgggtcgcttggtcttaggagcgtccaagctgcagagcccagtagacagaacctggatccagcgcctcactttacaggaggggaaactgaggcacaagcatgtgctacctggctcgggggccagcaggcagccttttcccttctgtcacctgccctagggatggaccgccccatctgccagccttgactggagcctccctggtggatgtttaccgcacacctactacgtgcagggtggtgcagctggcgagagtcccctctcctgttccacagaccggcaaggttcccctgagccctggggcaggcaggacctttggctggaggtgggtgtgcagggcagggtctctgaggggagacctcagactgtggacttgcgggtggacgcttctctctgtcggggcctcccgtgtccagaagatgttgaacagcatctgaggcttccacccgctgaagccgaggaacagcccccagctgtgacaacccaaaatgcctccagacctggccccatgtcctccagggggacggaacagcctggtgtagggcagggtcccctgagcaggagtggcacctgttcctgctcataccacagacagctgagctggctgtgcccaagactccctgcacccaccaaagccactggatacaggcacgatttgcatcttactctcttaagtcaggtttctggagatggctgtcccaacactggaatccagcctgtctacagcaagggagaaagaggaagctgatgttgggctgagaggggcaggcgttacagggtaggtctcacaaatgccgacgtgacaggcagggcttctgagggggcttcagggaccagcagggaggcgagactcaggcactgacccgcagagagcatggccttggacgcacagtggtgacagcagcctccaagtgtcccccgtgccctcaggcatgagggacagaagcttctggggcccctgcctctttcctgcccatcccctggtgaaggaaaatcgcctctgataggaaaagctggggccagactccctctccctgcattagtgtcgccgtcctgcctgtgaggtccccgggcccagggcacctcccgggacacccgagtggtgatgcacgaccctcagtcctggggcttaggacctctgggtgcccccgcaggtccgtcctggagtcacttcacagtcactgcaaatgggcaccacagcccactttccaacgccccaactttccacacccaagcagctccttgtccctgccaatcaatgcccggtgatgacaactgttcttttataaacaccacacatcttctaatgctttcatgttaaaagcgggagtggatcccacattcacctaaaggctcaggtagggactttttttgcagaaaaccaatttcttgtaacaagtactggaacctcattgtagccttgagtcctcactcctccttttgttctaagtctgggtctgagaagtgcaggcctcacacagctgtcagttccaagtgaccagggctgtaacaggtcctggctgaccctgggaatgtcaggggattctgggaagtaagaaggaggggcatttgcccatagccccggggcagacaatgtgtcccgagggccaggccaggctgtctactccatctccctggggcgagtgcacctcgggtcacctggcagcatcctttccagcccttctggagacagtcagcagctgattcattccgggaaccagcatggcaggtgccggggctggtcagggcccagggctgtacccctcagcactggaccaccccgtctcctgcccccttgggactgttgggctccgaggagcctggcgctggggtcggaggtcttcatcaggaccctggggaccctcagggttgagtggggtggggctgctgagggtggtgggggccgggggagccacctctcactttggggatcattgctgaggtgagaagggggactgtggccaccaggtgataccctctccatgcacctaactgctgctcaggactctggggaccgtgttgccaggcctgcgcctgctggacatgggcgtctccagccctgctgggctgtgtctttctcgctgcagagccaagagccccggcagcccctgtagccaaacacggccctggcacagcctttcttctggcaaactccacccgtgcgtcttccaaaggtggctcaacttttcaccggaacagccgagggacattgttcctcccagggaatgtggcagaggacactgaagcccagtggggacttccgggggctcctcggtgtggacggctaactacacttgtgggcacacacatgagtgggtcctgtggcttccgggcgggaggcaggttgggagcgttcagggcagaagagctcctgtgaccgtgtcccctgcaaacagcctcgcgtgaccccagcagcacagaggccgtcctggaagagcggacgcccagtcttctttttaaaccaaacacccttcggtctcaggatcccgcatcccacgggaagacccacagtgggtctggggtactgggaagagcctggtgctgaatcccgcacgctccgggtagagacagcccatcaccagtcccttcctgtgggtgactggcagtgacagcggggagcccactcacttggggacatttgcctttggtgtggatgacgcttttgaaagggcctcattccaggatcacagccaacgccagcaggttctccctgggatccagcagtggtccttctgggggctgccccaagtgctcccctgcagtctgggagtccatgctcaagctgccacctggcctctcacggtggcgtctcacggaagccctgtccacgctctgggcggtgagctccggtcaaacgtggccagtgagctctgtctccggactcacagcccaggcacctgcatagctgtgttggaggcatcggtccctgcacacccagcctatggccaccgccacgaccacaagcaggcacaggacagccaggatgctccacgtggccgcgtttttctcgccggtactgactggattctctgtgatcttgtctctctctccgatgtcatttcctgtctggctgccgacagtcaggttctgctgcagaagcacgttctctatgcagcagccaatgttcacgctgggggtccgtgcgatcctcagcacgctgaccacgtcatacaagccccgcatgttcaagaagacggtgtcattctgcagagcctggtccagcaggctgttgtccgtcttattgatccagtacacgttgggcctggggtagccgtttatggatgtacacgtgaaggtgagctcatcctgggaggggctgtggggggcgctgacgacgggcacgctgaagtttgctgccacatgcagtgtaacctcaacgctcaaaacctcctggaatcccagggattggctcaacaccaggcagtgaaacttctgctcgtcctggggggtgacgttgaacaagcgcagggagaagtcgccccgcagcatgccggccggtgacatcagggctcggttccggtagcggctgtccacgttttccaaggagctgttctgtgggatgtggtaggtcaccacggttttcgactcactggtttgccaatatacgtaaacatcatttaaatcaaaacggcttccttcagggcaagcgcagctgagctccacgtcgctgcctaccatcgctctgacttccttctcctgagtatcagctcgaaggctgctgaagagcaggaagagcagtccaggactggaaaaaacaaccagaaaggcaggtgaggcggggccaccagggagttacctgtatcttccaaacaggaacaggctggttcccatgagcaggaggtagttaagcccatcacagaaatgtgaaggcagagccaggagcctgcctgcctctgttctccatgggaattcggggtccggggccaggaccaccaccctcctgcccagcacagcaagtccgaggggctggcagcctctcaccactctctagctctcgcggtaacaaatccccagaaacacagtgatgctggcgtgaggatgaaggggagcgagggacgccagtgaggctggtctagccttcctgcccagccgcatggtgcgggcggagacctcgggccgcggagacctcggggcgcggagacctcggggcgcggagaacttgggccgcgggagacctcggagaggagcaacctcggggcgcgggagatcggctctaactgc

SEQ ID NO: 14067 - RNA, 2846 nt, Homo sapiens
  source 1..2846: mol_type = other RNA
gctgggattacaggcatgagccaccgcacccggccttggctttccatttctgcaaaaccacaggccactgctgccacttgctctgtggagatgtaccttccacttattaccaccttcttctcaaaatggcactcacggtactaacttttggagatctccagaggcgtcagttgcacctctggaagtaagatgatttccctgccccatacttgccaaagcacttttttttttttttttttttgagatggagtctcgctcttgttgcccaggctggagtgcagtggtgcgatcttggctcactgcaacctctgccttcccaggttcaagcgattctcctgccttggcctcctgaatagctgggattacaggctcccgccaccacacccggctaatttttttttcgtatttttagtagatacggggtttcaccatgttggccaggctggtctcaaactcctgacctcgtgatccacccgcctcggcctcccaaagtgctgggattgcaggcgtgagccaccacgcccggctagcacttccctttttaagctagtgctggcatgccaccttcccctcaaagcagagtcaacttccttttgtttgagagttttgtactggcctctgtaggcccttttcaggatacaaaataaagtgcccttcagcatccacatgcgagtgggttgccttccagtgtcagatctgtgttccagagtttggtcaatgcatctttacaagaataaaaccacatgcctacacacacagacgagcctggaaatggctttctggacagggttacttgttatcttgacacttcccctaaaagaaattactttcttggtgtaagatgattaggacattgaatgacctactctcaacttctggaagggcagcttgttttgtccatttttcaatgagggagtgggaagaacccaacattttcagttacaacaataagattttgtttttttttttttaaaaaagggtcctatgtggaaatgagtgggacaatgataaaaataaacaaataattaaaattccaaatcaaaacataactcctggccctgagatccccagttaatcctctaagaccacaatctccacattgtgaacttgatgctggtgttcttccatctcagccacaactttctcctcagtcctcagctctgtctccaagatgactgctttgccctcagtatcttcagcttctgggtccggggctggatcaatctcaatgatggtctgcccatcctctgaggtgctttcaacagcctgaattgccgaggttaggccggactccatggccaccaattccacagggctaaccatggtggtcatgttgcccagtgtactcccatcctgcatggcagtagagctcagcagcgccaagctagatgaagggtggatggtcactgtgtctggtgagctgctcttggcagaggagaccactgtggcatagcggaagagctgagggccagaaggcagtgtgtggacagtcacaggactggagccctggctgagggtggccactggaatattgcccatggaaaatgactgacccactggggtgatggtgatgggtgagatgactgtgaactgaggctgctggacaggaggagaagggctcaagacagtggtggaggctggccgctggagccggggcctttttggaggcttaggagtgctcacaggcatcagtaccacattttgaactgtctgagatttcagcctgtgatcctggccttgcttcttctgctcctccaactggcgttccaagtctgtcagagtatagagaaactgttcttctccctgctctacttggttccttctgttgtctaaaaccttcttgactgtgtccattaggccaaatgtgtgtgctacattgttgagaacagcagcatctgtgacttggaagggagcctggatgagccgctgctgaactcccctgagtagctcctctatttccttctgtatattgcagacaacctcttccatcagccctacatcagctattcctttccagaacatcaaagtgtcctctgaaatttcctctgagtctttctttacaccctcctccgtggccatggtgacagcagcggtgagagctgagttccattccagccctgcctcttccatgctctcttctgagatggcaatctgcgtgatgctaccatcagccgaagtgggtgtctgcaccacacttgtctgctgtcctggcactggagctcttgcactgctgatcagaagatcaaatttggtgcttctgcaggtattggagcaaactttgtcatgttggtaaaaatcaatctgtccggagtccatcattttcctgagcatgatcccacccagacgaatagctctcttccagtccttcagagtggacttgccagccagatgaacaaagtgcttggggctgatcaactgatcattgaacttgacacacttcacgtttattcctggacatacaaacttcttccagaggaggatggctttgctctccccacaagttatggggtaagcaatttccatatcctcatttgcttctatagtgcctgtatcaatcccttcttcaattttgtgtatcgtgtgagtttctactgctacaactgccgtgttgttctccgacccagcttcataaatcccttgttgcacaggctgtaactgcaaaatcacttgggttttagtgtcttcaggattctccccttcatttccttcagtaggtaccacaaccacatcccccactgggacactcacttctgcattagccatctttcacatgaagtcagatagctgggacgtctccgtcgggcgggcgggcggcgagcggccagggcgggcaggcgacggagcat

SEQ ID NO: 14068 - RNA, 2849 nt, Homo sapiens
  source 1..2849: mol_type = other RNA
gctgggattacaggcatgagccaccgcacccggccttggctttccatttctgcaaaaccacaggccactgctgccacttgctctgtggagatgtaccttccacttattaccaccttcttctcaaaatggcactcacggtactaacttttggagatctccagaggcgtcagttgcacctctggaagtaagatgatttccctgccccatacttgccaaagcacttttttttttttttttttttgagatggagtctcgctcttgttgcccaggctggagtgcagtggtgcgatcttggctcactgcaacctctgccttcccaggttcaagcgattctcctgccttggcctcctgaatagctgggattacaggctcccgccaccacacccggctaatttttttttcgtatttttagtagatacggggtttcaccatgttggccaggctggtctcaaactcctgacctcgtgatccacccgcctcggcctcccaaagtgctgggattgcaggcgtgagccaccacgcccggctagcacttccctttttaagctagtgctggcatgccaccttcccctcaaagcagagtcaacttccttttgtttgagagttttgtactggcctctgtaggcccttttcaggatacaaaataaagtgcccttcagcatccacatgcgagtgggttgccttccagtgtcagatctgtgttccagagtttggtcaatgcatctttacaagaataaaaccacatgcctacacacacagacgagcctggaaatggctttctggacagggttacttgttatcttgacacttcccctaaaagaaattactttcttggtgtaagatgattaggacattgaatgacctactctcaacttctggaagggcagcttgttttgtccatttttcaatgagggagtgggaagaacccaacattttcagttacaacaataagattttgtttttttttttttaaaaaagggtcctatgtggaaatgagtgggacaatgataaaaataaacaaataattaaaattccaaatcaaaacataactcctggccctgagatccccagttaatcctctaagaccacaatctccacattgtgaacttgatgctggtgttcttccatctcagccacaactttctcctcagtcctcagctctgtctccaagatgactgctttgccctcagtatcttcagcttctgggtccggggctggatcaatctcaatgatggtctgcccatcctctgaggtgctttcaacagcctgaattgccgaggttaggccggactccatggccaccaattccacagggctaaccatggtggtcatgttgcccagtgtactcccatcctgcatggcagtagagctcagcagcgccaagctagatgaagggtggatggtcactgtgtctggtgagctgctcttggcagaggagaccactgtggcatagcggaagagctgagggccagaaggcagtgtgtggacagtcacaggactggagccctggctgagggtggccactggaatattgcccatggaaaatgactgacccactggggtgatggtgatgggtgagatgactgtgaactgaggctgctggacaggaggagaagggctcaagacagtggtggaggctggccgctggagccggggcctttttggaggcttaggagtgctcacaggcatcagtaccacattttgaactgtctgagatttcagcctgtgatcctggccttgcttcttctgctcctccaactggcgttccaagtctgtcagagtatagagaaactgttcttctccctgctctacttggttccttctgttgtctaaaaccttcttgactgtgtccattaggccaaatgtgtgtgctacattgttgagaacagcagcatctgtgacttggaagggagcctggatgagccgctgctgaactcccctgagtagctcctctatttccttctgtatattgcagacaacctcttccatcagccctacatcagctattcctttccagaacatcaaagtgtcctctgaaatttcctctgagtctttctttacaccctcctccgtggccatggtgacagcagcggtgagagctgagttccattccagccctgcctcttccatgctctcttctgagatggcaatctgcgtgatgctaccatcagccgaagtgggtgtctgcaccacacttgtctgctgtcctggcactggagctcttgcactgctgatcagaagatcaaatttggtgcttctgcaggtattggagcaaactttgtcatgttggtaaaaatcaatctgtccggagtccatcattttcctgagcatgatcccacccagacgaatagctctcttccagtccttcagagtggacttgccagccagatgaacaaagtgcttggggctgatcaactgatcattgaacttgacacacttcacgtttattcctggacatacaaacttcttccagaggaggatggctttgctctccccacaagttatggggtaagcaatttccatatcctcatttgcttctatagtgcctgtatcaatcccttcttcaattttgtgtatcgtgtgagtttctactgctacaactgccgtgttgttctccgacccagcttcataaatcccttgttgcacaggctgtaactgcaaaatcacttgggttttagtgtcttcaggattctccccttcatttccttcagtaggtaccacaaccacatcccccactgggacactcacttctgcattagccatctttcacatgaagtcagatagctgggactgcgtctccgtcgggcgggcgggcggcgagcggccagggcgggcaggcgacggagcat

SEQ ID NO: 14069 - RNA, 2879 nt, Homo sapiens
  source 1..2879: mol_type = other RNA
gctgggattacaggcatgagccaccgcacccggccttggctttccatttctgcaaaaccacaggccactgctgccacttgctctgtggagatgtaccttccacttattaccaccttcttctcaaaatggcactcacggtactaacttttggagatctccagaggcgtcagttgcacctctggaagtaagatgatttccctgccccatacttgccaaagcacttttttttttttttttttttgagatggagtctcgctcttgttgcccaggctggagtgcagtggtgcgatcttggctcactgcaacctctgccttcccaggttcaagcgattctcctgccttggcctcctgaatagctgggattacaggctcccgccaccacacccggctaatttttttttcgtatttttagtagatacggggtttcaccatgttggccaggctggtctcaaactcctgacctcgtgatccacccgcctcggcctcccaaagtgctgggattgcaggcgtgagccaccacgcccggctagcacttccctttttaagctagtgctggcatgccaccttcccctcaaagcagagtcaacttccttttgtttgagagttttgtactggcctctgtaggcccttttcaggatacaaaataaagtgcccttcagcatccacatgcgagtgggttgccttccagtgtcagatctgtgttccagagtttggtcaatgcatctttacaagaataaaaccacatgcctacacacacagacgagcctggaaatggctttctggacagggttacttgttatcttgacacttcccctaaaagaaattactttcttggtgtaagatgattaggacattgaatgacctactctcaacttctggaagggcagcttgttttgtccatttttcaatgagggagtgggaagaacccaacattttcagttacaacaataagattttgtttttttttttttaaaaaagggtcctatgtggaaatgagtgggacaatgataaaaataaacaaataattaaaattccaaatcaaaacataactcctggccctgagatccccagttaatcctctaagaccacaatctccacattgtgaacttgatgctggtgttcttccatctcagccacaactttctcctcagtcctcagctctgtctccaagatgactgctttgccctcagtatcttcagcttctgggtccggggctggatcaatctcaatgatggtctgcccatcctctgaggtgctttcaacagcctgaattgccgaggttaggccggactccatggccaccaattccacagggctaaccatggtggtcatgttgcccagtgtactcccatcctgcatggcagtagagctcagcagcgccaagctagatgaagggtggatggtcactgtgtctggtgagctgctcttggcagaggagaccactgtggcatagcggaagagctgagggccagaaggcagtgtgtggacagtcacaggactggagccctggctgagggtggccactggaatattgcccatggaaaatgactgacccactggggtgatggtgatgggtgagatgactgtgaactgaggctgctggacaggaggagaagggctcaagacagtggtggaggctggccgctggagccggggcctttttggaggcttaggagtgctcacaggcatcagtaccacattttgaactgtctgagatttcagcctgtgatcctggccttgcttcttctgctcctccaactggcgttccaagtctgtcagagtatagagaaactgttcttctccctgctctacttggttccttctgttgtctaaaaccttcttgactgtgtccattaggccaaatgtgtgtgctacattgttgagaacagcagcatctgtgacttggaagggagcctggatgagccgctgctgaactcccctgagtagctcctctatttccttctgtatattgcagacaacctcttccatcagccctacatcagctattcctttccagaacatcaaagtgtcctctgaaatttcctctgagtctttctttacaccctcctccgtggccatggtgacagcagcggtgagagctgagttccattccagccctgcctcttccatgctctcttctgagatggcaatctgcgtgatgctaccatcagccgaagtgggtgtctgcaccacacttgtctgctgtcctggcactggagctcttgcactgctgatcagaagatcaaatttggtgcttctgcaggtattggagcaaactttgtcatgttggtaaaaatcaatctgtccggagtccatcattttcctgagcatgatcccacccagacgaatagctctcttccagtccttcagagtggacttgccagccagatgaacaaagtgcttggggctgatcaactgatcattgaacttgacacacttcacgtttattcctggacatacaaacttcttccagaggaggatggctttgctctccccacaagttatggggtaagcaatttccatatcctcatttgcttctatagtgcctgtatcaatcccttcttcaattttgtgtatcgtgtgagtttctactgctacaactgccgtgttgttctccgacccagcttcataaatcctgttgtaaaagtgtccatcgataaacaaaccttgttgcacaggctgtaactgcaaaatcacttgggttttagtgtcttcaggattctccccttcatttccttcagtaggtaccacaaccacatcccccactgggacactcacttctgcattagccatctttcacatgaagtcagatagctgggactgcgtctccgtcgggcgggcgggcggcgagcggccagggcgggcaggcgacggagcat

SEQ ID NO: 14070 - RNA, 3292 nt, Homo sapiens
  source 1..3292: mol_type = other RNA
gctgggattacaggcatgagccaccgcacccggcgtggggtcatgttcttaacctttcttgtgcttaaggttttttgagattcttggatttgtagcattataattttcatcaaacttggaaagttttcagtcattctttaattttctttgagtctttaaaaacaggcttactggaatttaattcacatcatacaatgcacacatttaatttgtatagtgcaatgttttgtagtatatttatagagttgggcaaccatcacaacagtcaattttcaaacattttcattaccccaaaatgaaacctgatacccactggcagtcactttccaattacctccaacttataagccctatgcaatcacttatctatgttctatctctacagatttgcctattctggacttaaaaaaaatagtcatgcaatacgtgtcttctgtggtttaaaaaacagaatgtactgtctcacagttctgggggctaggtaactgatagcaagatgttagcagcattggtttcttctgaggcccctctcctcggcttgtagatggccatcttcttatgtccccacatgatcttctctctgtgtgtgtctgtgtcctaatctcctcttcttgtaagaataccagtcaggttggattaggtccactcatggacctcattttaccttaattatctgaagaccctatctccaaatacagtcacattctgaggtgctgggggttaggacttcatcatatgaatttttgggaaacacaattcaacccataatactaggcagtgaggacactgaattcattatactatttactctatttttgtgagagtttgaaatttttcataatagaaggttttaacttttattaaattagaaaattgatggaagagaataataaagttaagccagtatgaaccactgtaatagctctagaaagaaatacaatcacttatctttaaaaaaaaaatgacttgataatccataggcctattagcagaccaccttttacattcctgaagggtgaattttgtcccctcaaattcaaatattgaagtcctaccacccagtacctcaaaacatgactgtatttggaaatagggtctttagataactaaggtaaaatgaggttatacgagtggatcctaatccaatctgaatggtatccttataagaaaaaaagattagggcacagacacacaaagagggaagaccacgttgggacacagggagaagatggccacctgcaagcccaggagagaggtctcagaagaaaccaaccctactgacatgttaatagcagctgtagagcctccagaactgtgaggcagtagataaggtacctcagcctccaatgtctaagaaacccaagatcatatccagtccaaagggcagtcagaccttccctatgttaggcattagatagaactggagtctctttagtacaccactgatttaacttttgctgacatttaatattgccatttaagtttaatctttcacaatattacaagtatatcacaagttatacttgccgagtaaagcaacacaagtgaccttaatggtctgtatcatggcataggctgaaatattagagggaggacaattgaatatctccatgctagggtcagccccaacatgtaaatatcaaagttacagccattagcttttaggtttttttggttcacttatgcaatttcttattaatattcctccaagagaactgaggatatttccaacacaccatggagtcagaacacccaatgaatcaagatgaaataagataaatatccaaattagctcaatgggagaaaagaggttaatagtcacagaatcatagaatttagagggctgacttccatttatggcaatatagtaaattaactgagaaccctcctatcaaaaaacacctggaaatgatggacaaaatataataaacatgcttttaaatatataactgaacatgcaagaaagtaagagaaatccctcggggcaaagccagaaatgaaacagaaatgcagctcagactgccctgataaatgttgctggacttgataactgaggggctactattttaacagccatgtgaggacaggagataaagccttgaatctatagtaggaagctagagtgtaagttatctagtatcagcaccctcaaaggcttatacttcagtaaaagggtagattaggaataacatccacccactggcaaagaggtgtgacaagagagctttctggtctcatcttgtcctctaggttacattgtctttaaaaccaatattactctgagaattctaactatgaatcattttctcctgcatttgcagtttaaattcatactatctttgtggtctgtgaatctcacctctggtatgcctgagaggaagaaatgctttgagggacacaactttaacccacacctccaaaatctcaacagatgaggctccaccagacatcattagctcatcatcactaagacaagtgagaagattcgagggttggacccactcatatgtaactgaatcatctgaaacccagatattttaaatgacttacccaaaagttccacagcatttaattggcagagacagaccagagctcagggcttatgagttgtctgtgaattatttactccttccagcaatctgcctctttccatatagaagttctttctctggagaatctaagggaaaaatcaggttcaattgtctttatttatttatttatttgtttgtttgccttgagacggggtctcaccttgttgtccaggctggagtgcagtggcccagtctcagctcatggcaacctcctactcctggattcaggtgattctcctgcctcggcctccagagtaacagggattacaggtgcataccaccacatccagctaattttgtatttttagtagaaatggggtttcaccatgttggccaggttggtcttgaactcctgacctcaagcgatctacccaccttggcctcccaaagttctgggtttacaggcatgagccactgtgcctggcctcacttttcaatataggattgttgattttgaagacaattgaggccaagcatcgtgggtcatgcctgtaatgccagcattttgggaggcagaggcaggcagatcacctgaggtcaggagtgcaagaccagcctgaccaacatggtgaaacctcatctccattaaaaatacaaaaactcactttgggaggccaaggcgggcggatcaagaggtcaggagatcgagaccaccctggctaacacggtgaaaccccgtctctactaaaaatacaaaaaat

SEQ ID NO: 14071 - RNA, 649 nt, Homo sapiens
  source 1..649: mol_type = other RNA
gctgggattacaggcatgagccaccgcacccggcttcattttcctcatctttaaaatgaaatgatgatagccatcctctcataaaaatattaggattaaatcacgtaaagcatgattcttgtcttgtctccttgttcccaattctttctgtctggtttctattttattgtgcctgttcttacctgtccttcccttttgtggagaaggggagagcagagagccccagcagagctatgctgtatcattgctatgtagatggagctcattaaacacccctcgattgcttgaatacatgggagatccactcttagaacatttagggacaatatttcctgtcccctcatgtcaccttgatacttcccctgggtgaaactggaagtttttgagcaggagtgacaagttctgagttccatcactctgagagctacgttgagagtagagtgcaggggccaaggtcagacggaaggagaccagtcagaggctgctgttataacccaagtggtgatttggccaggtggcagccagtgaaaaatacagccaaaaagatgacacagtactagcaaataagatgtactaaaactacataaaaattaaaagtttaaaagaatgatttaaagaaatatgaattccaatattctctttcccaaac

SEQ ID NO: 14072 - RNA, 2198 nt, Homo sapiens
  source 1..2198: mol_type = other RNA
gctgggattacaggcatgagccaccgcacccggcttgcttcttattcttgttatgattgtttctagtcccaggtagacaaacaacacggccttcctcagcctctacccgagtcgtttcagaagagtgtgagccatgagaaatcagagctgttattttctggttgaaactgacactttaggctactgttttcatttgctttcaaatgattcagagaagaaagtacttatggaaagagaaagaaactgcaaaaggtggcaaatgctagccactggttgatctgaatgaagaatatgtagatgtccattgttttgccttttaattttctgtaggcaagggaaagataggaaggagggaaggtgcaggcatttcttatcaattcatacctgactaggatcacctgtaggtaacttaaagtactttttctggaggttccagtccttctacttcatatgttttattccatcattcgtggaattgccagttgttcaaaataaacctctaaatgatcatcgtaagacatttcatcatcaatatcatccatactatggatttgttttaaaaatgaggtaaaagtcattaagaaaatgaaagcacaaaagtctatcaaaattacaaaaacttaaaactgagtaaacaaaacttcagaaagaatgaaaacaattggaaaataacttcaagaaaaaaatgtaaaatggaaacaatacaagaacaatttgtgccctctgaaaaacagaggttaaagtcagaatttttttgttctttttttttttttgagacaaagtctcactctgtagccaggtgctggggtgcagtggcatgatctcggctcaccgcaacctccgcctcctgagttcaagtgattctcctgcctcagcctcccaaatagctgggactacaagagtgcgccaccacgcctagctaatttttgtatttttagtagagacggggtttcaccttgttggccaggctggtcttgaactcctgacctcaggtgatccacccgcctcggcctcccaaagtgctgggattacaggcataagccaccacgcccagccaggaaagtatttaaaaacaaattaagcaaagattataaaagtttttggagtaacacatttcccgaaatgatcacgatccacatcaagtctgagccatgttgacatccccacgtcggggcccttcctggtggtcgaggaatcttcagaggtctctaaaatatattaaaaatgtcccaacatttcaggacattccaccggcttttcttgctgggcttcctggttttcttcttgggctttctggttttcacttcctcttccactttggtcttttctgttgcttcttctgcaggtgcagaggaaggacttgctgacatctgctggtggctgcctgtaatggtggagtcttccaatttctttgccggtgtggctgggtccacctgcatcatgtgaacccctgtggcttcctcagagactgtctgccctggcagatgctcctccaggtcttccaggtcaccacgttgtggaactcccaaggatgtcttcatcgcctcttggtacttcttccatgtgctgtataggtggagctcccgtagtcgccgtagttgccgtttcatctcaatgtctctctctgtgtctttgtccaccatatgaacgcccaggacatcttcagatgaagcttcctgcaccaggtcctcatcgtaatctggattgtaagttttaagaatcttctttttaagttccaaaatttggtgtcgaattggttttttttttttcttttctttttttggagacggagtctcactctgtcgcccaggctggagtgcaatggcgcgatctcggctcactgcaaactgcgcctcccgggttcacgccattctcctgcctcagcctgccgagtagctgggactacaggcgcccgccaccacgcccggctattttttttttttttttttttgtatttttagtagagacggggtttcaccgtgttagccaggatggtctcgatctcttgacctcgtgatccgcccgcctcggcctcccaaagtgctgggattacaggcctgagccaccgcgcccggccgactcacggtattttttgatagaggaatgagttctctcattaggcacctcctataatgtatataacatcatgttttaaacgtgtaggttaaaaataacactgtgtatgcttagcttggtga

SEQ ID NO: 14073 - RNA, 632 nt, Homo sapiens
  source 1..632: mol_type = other RNA
gctgggattacaggcatgagccaccgcaccggccaacatgtgttttcagcggtgtgaccctgtgcaagccgtgttatgtctctgtgcctcagtttgcttgtctgtaaggtgcaaaggctgcgagttgcaacttccgagggtcgaggtgaggggttagcagatcatcaggtggcacacagtgggcactgcggaagtgtgtgttgctgccactgttggcaggaatattgagcctgccccgtgcctcctcaggggccctgtgggtttgcgtcgtcctgagcccccacatcatggtcctcttcccaggagagagagggagtggggcagagcaaagcagaccccagtccttggctgttcttccaggactaatcccaacttgtctagccaggaaagagcgagtgccaagggcaggagcaatggcagcccaagtgggcaagtgaagtaaaatgcttaaaacacctgcagtcctgggctggtctggcttggccttctgctagctatgggaccaaagagaggatgagagaggaaaaaaggaggaatcaaacagaaggggaaagtgagatattgaggagagagaaacaagtgaagagaggcagagatggatggagagagggagaggcagacagaggagcaga

SEQ ID NO: 14074 - RNA, 535 nt, Homo sapiens
  source 1..535: mol_type = other RNA
gctgggattacaggcatgagccaccgcaccggccaacatgtgttttcagcggtgtgaccctgtgcaagccgtgttatgtctctgtgcctcagtttgcttgtctgtaaggtgcaaaggctgcgagttgcaacttccgagggtcgaggtgaggggttagcagatcatcaggtggcacacagtgggcactgcggaagtgtgtgttgctgccactgttggcaggaatattgagcctgccccgtgcctcctcaggggccctgtgggtttgcgtcgtcctgagcccccacatcatggtcctcttcccaggagagagagggagtggggcagagcaaagcagaccccagtccttggctgttcttccaggactaatcccaacttgtctagccaggaaagagcgagtgccaagggcaggagcaatggcagcccaagtgggcaagtgaagtaaaatgcttaaaacacctgcagtcctgggctggtctggcttggccttctgctagctgtattcccagctactcaggacactgaggcaggagaatcc

SEQ ID NO: 14075 - RNA, 3920 nt, Homo sapiens
  source 1..3920: mol_type = other RNA
gctgggattacaggcatgagccaccgcaccggcctagaatttcaactactaatttacattaagcttttaattatgtttaaagtgcttttcctatcagagtttagcctcttagatgtagtatgtgctagacacttgaagttttgtttgttacagccctttcttagctatcctgctttgtatgcaaggatgttttctagaaatattgaagggtgagaaaacaaaactatcagccattgaaaactatatttaaatttggatacttttgtacatactaaattatcttaaaaaaatagaaacgccatatttctttcccatggcttgtctttccaaataatgtgttgtttttaagtctgtcacaattagacctattctcccctagcctgtttggtttgatacatgccacttatgataacataaaaggagaaagaaggcaggtgccaattatttactcaggtaaagaagagagaaaaggcaccaaaggtttttttttttttttttttttttttttttttttttttttttgagatggagtatcactctgtcacccaggctggagtacagtgacgtgatcttgtctcactgcaacctctgcctccccagttcaagcaattctcctgcctcagcctcccgagtagctgggattacaggtgcctgccatcatgcccagctaatttttgtatttttaatagagacggggtttcaccatgttggccaggctggtctcgaactcctgacctctggagatcctccctccctggcctcccatagtgctgggattacaggcatgagccaccgcacctggcccaaagcttgattttctaatttctagggttcacactacttctattattacaaaaatctcaaattctatgcacctagtggctagaatgaataattaaggcctctaggaacttggaagaaggacagattggagttgtctggaaaattttttatggaggacacaggatctgacccgggagttgaagactgggtaggacgttcattaatggagaacaggagggaagtctcttggaaggattaatgcgagcaaaggcacaagggtgtgcacaaggatgtttcatcgagtagagtataaaggatttgtgggaaataagacaggattagtaaattggggccaggcaatggagtgccttaaagaataggataagtagttcaagtttaatccttcctgtaagcaagtttcctttaaaatatgtttgagagtgataaaatcaaattagacttacagagtaaacacatatgagcgtgtgtgtgtgtgtgtgtatttagccaaaaccaaaagcttgtcaataactatattatgtaaaacttcttttctataaaaacagcatgctgtctcccattgtccctctatatatgaaaacttgctgccaggaagttttcatatatgcagggtttactttcccattacttttcctagtgacacttagttttcaccatgttctgtggcttacgtgttctgcccctcacaggtacccctatagaaagaatactccaaaacaccaagggagtcaccaagagagaaagccaggcagggtgggaaactgaaaatctccactgattctgcagagaagctctaaggaacaatccttccatttcaaagcatcagaagggccaggagctcaattcatccttcacatttccataggatgaaacattatttgttccctttaagatactatgtgatgaattaccgcagaagagatggaaggagaaaaaaatgggaatacaatagttaacacttctgttatatttattatttaccagaagaaaacaataataaagcaaatgtttaaaaaattttctttaacttctgcttcgggaaatatgactctaaatttcacctgagtcactcaaattgattgcaagtagaaaatattgcctctaaatattatattttatctccttccaccttcctcttcagcccctacttcttcatggcccaaacattctgccttttacaaatacccttatcagatggtagcattgtttccagttctgccacgtggatcctaaagtattgctgctgacatagtctccatgctgtaatccaagagtcactatttccatttcttgttcttctagatggctctgttgcctcttacgccagttcttttggcagttgcacaggtttaagataggcgacactgctgtgacgaatgtcgtttagcagctgatctctgggagtgatttccaccaatgggggtggcctgtttctcggcactggcttgagcgttttgatgacatctttgaggttggttttctcgggtggttctctggcttccggcatccgagatttgcgctggattctcttcagcttcaccacccggaaggagtcagggtctgtcctgtacttcggggcctgcgatggctttttcatcatttcactgcgttgactaaaggggacattttgggggttgggaggccgaggtggcggtggctggaagaattcctgcattctggaatctggcttgggtcctcccaacagctcccacatcccagggggcagccccaacccattctctaacatggctatcagcttcttctgttccttgagttgctgctgtttttgctcttcctgtcgtttctgcctttgtttatcctgattcctggtgagcagattagtgaccaccattctgggacccggaagctcaaaatggtagcccatcttcaggagagtgttgtttgccttcaaaagcctggctatttccatttcagcatggtgacccaacatgtgcctctgattgtgaaaccgaagctcagttagcgtctcattaaactggagacacctcatgatggccacaatccctttacctgtgatgaaattggactcgatgttgagagtggtgatgcttctattttcacgcaacatgttagccaaggcaaatgctacattctcatctgcacccacattggctaaactgaatgttttgatgtgcttgtttttcttcattgcattgacaaagtccagtaacatttctttggggatgttttcaatgttgttcaggttgagttccttcatgtcaggatcatttttcctaactctcctcaagctcccatccaggtctgtctggtttcctgaaggccttgtacttaccttcaaaaagctggtgtctagagctaacttcttaggatctaatttcgatatttttttctcactttgttcttgggcctctggtctgtctctctgttctttgaatgctttgtcagttacctgctggcagttgttctcacaatttctaatttgttcctttgctttgccttcctcttctctgttcgtttcttcactctcttcaccatcatcttctccttcgtcgtcatcatcatcatcttcttcttcttcatcttcttcatctgtttcttggatattgctgctgccctttgattctcttttatttgcaactatttcattattgagcttttcttttaaatactgggccatatttttattacgtttttctatttcttcatgctcttcttgagtcttttcctcggatttcacaaaggtgacaggaactcgttcctcttccagcatgcgcctggatgccttttcccaatacatataatcaacaagagatttatgattgaagtttcctgtcggtggcttgtcagtttgatctttctgaatcattcccacgggaaggctggggtcaggggccatgacttccatttccgactgcagttctttcagttcttcagcagacaagttggccaagatttcatcttcattaatctcctcatcgagaagttcttcttgatctgaatttctgctgtgctctgacattattttttctaaatattattttaccttgagatatttttttttttttcccaggaacctcagtggtttgctgagcagctaggagtgatcacagctaagctcttgccggatctatatt

SEQ ID NO: 14076 - RNA, 4014 nt, Homo sapiens
  source 1..4014: mol_type = other RNA
gctgggattacaggcatgagccaccgcaccggcctagaatttcaactactaatttacattaagcttttaattatgtttaaagtgcttttcctatcagagtttagcctcttagatgtagtatgtgctagacacttgaagttttgtttgttacagccctttcttagctatcctgctttgtatgcaaggatgttttctagaaatattgaagggtgagaaaacaaaactatcagccattgaaaactatatttaaatttggatacttttgtacatactaaattatcttaaaaaaatagaaacgccatatttctttcccatggcttgtctttccaaataatgtgttgtttttaagtctgtcacaattagacctattctcccctagcctgtttggtttgatacatgccacttatgataacataaaaggagaaagaaggcaggtgccaattatttactcaggtaaagaagagagaaaaggcaccaaaggtttttttttttttttttttttttttttttttttttttttttgagatggagtatcactctgtcacccaggctggagtacagtgacgtgatcttgtctcactgcaacctctgcctccccagttcaagcaattctcctgcctcagcctcccgagtagctgggattacaggtgcctgccatcatgcccagctaatttttgtatttttaatagagacggggtttcaccatgttggccaggctggtctcgaactcctgacctctggagatcctccctccctggcctcccatagtgctgggattacaggcatgagccaccgcacctggcccaaagcttgattttctaatttctagggttcacactacttctattattacaaaaatctcaaattctatgcacctagtggctagaatgaataattaaggcctctaggaacttggaagaaggacagattggagttgtctggaaaattttttatggaggacacaggatctgacccgggagttgaagactgggtaggacgttcattaatggagaacaggagggaagtctcttggaaggattaatgcgagcaaaggcacaagggtgtgcacaaggatgtttcatcgagtagagtataaaggatttgtgggaaataagacaggattagtaaattggggccaggcaatggagtgccttaaagaataggataagtagttcaagtttaatccttcctgtaagcaagtttcctttaaaatatgtttgagagtgataaaatcaaattagacttacagagtaaacacatatgagcgtgtgtgtgtgtgtgtgtatttagccaaaaccaaaagcttgtcaataactatattatgtaaaacttcttttctataaaaacagcatgctgtctcccattgtccctctatatatgaaaacttgctgccaggaagttttcatatatgcagggtttactttcccattacttttcctagtgacacttagttttcaccatgttctgtggcttacgtgttctgcccctcacaggtacccctatagaaagaatactccaaaacaccaagggagtcaccaagagagaaagccaggcagggtgggaaactgaaaatctccactgattctgcagagaagctctaaggaacaatccttccatttcaaagcatcagaagggccaggagctcaattcatccttcacatttccataggatgaaacattatttgttccctttaagatactatgtgatgaattaccgcagaagagatggaaggagaaaaaaatgggaatacaatagttaacacttctgttatatttattatttaccagaagaaaacaataataaagcaaatgtttaaaaaattttctttaacttctgcttcgggaaatatgactctaaatttcacctgagtcactcaaattgattgcaagtagaaaatattgcctctaaatattatattttatctccttccaccttcctcttcagcccctacttcttcatggcccaaacattctgccttttacaaatacccttatcagatggtagcattgtttccagttctgccacgtggatcctaaagtattgctgctgacatagtctccatgctgtaatccaagagtcactatttccatttcttgttcttctagatggctctgttgcctcttacgccagttcttttggcagttgcacaggtttaagataggcgacactgctgtgacgaatgtcgtttagcagctgatctctgggagtgatttccaccaatgggggtggcctgtttctcggcactggcttgagcgttttgatgacatctttgaggttggttttctcgggtggttctctggcttccggcatccgagatttgcgctggattctcttcagcttcaccacccggaaggagtcagggtctgtcctgtacttcggggcctgcgatggctttttcatcatttcactgcgttgactaaaggggacattttgggggttgggaggccgaggtggcggtggctggaagaattcctgcattctggaatctggcttgggtcctcccaacagctcccacatcccagggggcagccccaacccattctctaacatggctatcagcttcttctgttccttgagttgctgctgtttttgctcttcctgtcgtttctgcctttgtttatcctgattcctggtgagcagattagtgaccaccattctgggacccggaagctcaaaatggtagcccatcttcaggagagtgttgtttgccttcaaaagcctggctatttccatttcagcatggtgacccaacatgtgcctctgattgtgaaaccgaagctcagttagcgtctcattaaactggagacacctcatgatggccacaatccctttacctgtgatgaaattggactcgatgttgagagtggtgatgcttctattttcacgcaacatgttagccaaggcaaatgctacattctcatctgcacccacattggctaaactgaatgttttgatgtgcttgtttttcttcattgcattgacaaagtccagtaacatttctttggggatgttttcaatgttgttcaggttgagttccttcatgtcaggatcatttttcctaactctcctcaagctcccatccaggtctgtctggtttcctgaaggccttgtacttaccttcaaaaagctggtgtctagagctaacttcttaggatctaatttcgatatttttttctcactttgttcttgggcctctggtctgtctctctgttctttgaatgctttgtcagttacctgctggcagttgttctcacaatttctaatttgttcctttgctttgccttcctcttctctgttcgtttcttcactctcttcaccatcatcttctccttcgtcgtcatcatcatcatcttcttcttcttcatcttcttcatctgtttcttggatattgctgctgccctttgattctcttttatttgcaactatttcattattgagcttttcttttaaatactgggccatatttttattacgtttttctatttcttcatgctcttcttgagtcttttcctcggatttcacaaaggtgacaggaactcgttcctcttccagcatgcgcctggatgccttttcccaatacatataatcaacaagagatttatgattgaagtttcctgtcggtggcttgtcagtttgatctttctgaatcattcccacgggaaggctggggtcaggggccatgacttccatttccgactgcagttctttcagttcttcagcagacaagttggccaagatttcatcttcattaatctcctcatcgagaagttcttcttgatctgaatttctgctgtgctctgacattattttttctaaatattattttactagaaaagaagaataatcaaagatgatttttaaaaagaaggaaaaaagcctcaagaaggtcccccagttaacgagtgtcccaagttaacacacccttgagatatttttttttttttcccaggaacctcagtggtttgctgagcagctaggagtgatcacagctaagctcttgccggatctatatt

SEQ ID NO: 14077 - RNA, 7468 nt, Homo sapiens
  source 1..7468: mol_type = other RNA
gctgggattacaggcatgagccaccgcaccgggccagtttcctgactttttattttcagctataaaacaattatgagagccaaaggagccaggatcaccttccaaaacattttgttttgtccttctctaatttatgaggcattctttcttctcaaagcaggatattacagtgcagattaaaactggatattaaagttaatggtgacaaattattaagtagtttgaagaaatccttagaatatcagataaagagagacttaatggcagaagaagaagtctactggggttcaaagcttaggttttatatttctgccatggtatctcaacactttctctgggatagtacgatgccctaaaaaatacctgtgttaggcagacaagtctaaatctcctttctcaggacaataggacaaaactgaacttgaggcaatagttgaagaattttaccccgtttttcaagtttaattttcttgagatcagaaaagtaaaattagaaagtagaatccttcatgtaaaaaaatatatgcgtatcacaatttattaaactctaacatctaagagcaaaaacaccaggattaagtaagaacatgcatgaactaaaatttagatagatattcaaagtaagttaaatttaccagagtcctgcatctggcctctcccatgccattatcgctattttgcaatttgttttgttcaggaagcctctgattttaatatttaaagtgtcacctgagaagagtaacctcaattcttcatgttttctcaacaatcttagaggtgttggacatcattaataaaatatactaaattatcagagaacttaagaacgctaagattctgatgagttcctttaccattttcagtcactttctaaaagggatttaacttcacattatcaaataacattttacactaaaaacacaatttatatagccctaaaataatattacttgagagatctaaatgaattccaccaatgcaaacgaagtttatatactgtattagtaatttgataccaccgtattccatggagaaaaaggcaaagagaatctaaatatttagatctgtgaaagatactagaaaaaaatagatttttaaatgcttctgatcctctcaaaatactcttgattttgactctatagtctatagaacacacaaaaaactgtaaaatgcatttgggaagagatcacgccatactcaaagaaaattctacaaattttgacagcattaaaaaaactgacttaagatatattttgttattgagaaaaaagtgtgcacattcaagaacataggatgtgtaatatttgtgataaattaagtcatactttgtgcttatactatgccctttattcaggagtgcaaaacacttaatcaaaaagagcatccttcacatatttaaagagtacattgaggcacagaaagtttgcccaaggcaagatagaaagtcgggtttatagacacaaaatgatctagaattcttcatgtccaattccttaaaatacaaactgtagactatttgtaatgcctccatcttattttatcaaacattagtaattttactattataagtttatgcataagtactgtgtgataggtaatgcccataaggtttttatcatgttttaaggtaacttgtgcatggaataggaaaagttaatcaaatgtaatcaattcgcttttgctttttaacaaaacttaaataaatgagctatttgaggacagttctggaaattcttgccttgatttttctccaagattttagatatgtagttcacatgtgaacattaatatatgaacaattattttatttattggcctctagttctctttcctctcatgatctgtctcttagtgaattgactttctgattcattgaaagcaaaatgctaagaaggttttgtgcaagtgcaaaatgtttaatcttgggttcagtcaactagtctctgatactaacttgcttagttaagccaagatcaagaagtatgagaaagaacttgaaatatgataaagaatttgaaacagaatatgggataagtagtcaatatcagaaatgtgagacaataaaaacaagatatattccaaagcctaatcctaaatttaaatctacacttcattcaactctgaacctgaccttgaaacatggaagaagttactttacctaagcacactgcaccagtgtaaaaccaatgccaattttagctgctttatactgcttaatgtgtatatgtacacatgtattcttaaaatggtgattcttaaattgaagttctgaattcttttgagaatctaacagaggtcatgaaaacttgcttcagaaacacacatatgtaaagtacttttaagtgttgatcatgtactataaatcacagcattgtggatgcaatgggattagacatgaagaaaaattttatatttttaataaagactggttactaaccttaaggaatatacttagactctgaaagtaaaaggaaagtgcaatgaccatatttgttcattcatctgcctattttcaaatctaatgatgatttggttgatgcaaatatgtccctaatctaggctataaatgataaaaacaaaaatgtttaagttctaacttttgttagcagtatacatctaagaattttcaagtattacaaaatacttggaaggaaagactttaatataccactttcaaaatcctatgtacccaaaccagcaatgaagtggtgggatatataacgttaccttgggcaaaatttaagaaaataaagacacaatagctctaattttttttttttttttttttttgagacggagtctcgctctattgcccaggcttgcatgcagtggtgctatctcagctcactgcaatcactgcctcctgggttcaagcgattctcctgcctcagcctcccaagtagctgggatgacaggtgcccgccaccatgcctggctaattattgtatttttagtagagacagggttttgccatgttggccaggctggtctcgaactcctgatctcaggtgatccacctgcctcggcctcccaaagtactgggattacaggcatgatctaaattctttatacccttcaagggcaggaaaccagtatctctgaaaagcttgtttgttttaatacaattgaacatttcatctttccccccacagtaatcaaagcaaacattttatcattattattcttggtatatcaaagtaaattccaggaatgtaagaaagtctgacttggaaatattacatagaaaaaggctgaattaacacattacattttttagtttttccttgtaagtatacattgacatctacttatctgatagcagcactgctggttttgagtgagttttgttttgttttgtttccttccagagggaatgcagtatggcagcattttctttggaacaaattaagaagatagtaacaaataacagaagaaatacttctacacatatattttccatgggcaataaacagataagtatataattatgaaaaaatatgcctcaactatgctttttaaaatttctcaaggtatactggtttgtttttcttattcaaatataatgcactatcactactatctgtcccgggaaaaacaaaccctgaggtttgagttacctccttcagccaacagagtgatatcaagagtaaacttggattgaggtcaacctgtttgagccaatagagagttctgtagtatatctggttattttactaacgtatacatattctaggttataatcaagatactcattaaatattttctatcagagttttatatcccaaacaggttctttgatgatttatcatgctaccataggaaatttgaagaaataacaaattgtgtaacagaaatagacatgcaatataaaggacataaaagatacagcttgaccctggatttttcccttagaataattccttccataaataagactctatttttacatacagattcatcctataactggtcttggatcataaagttaatgacatagttgaaaaaatccagaccacacatttttgtggtcttttgtcaccccagaccacacacaaaaaaaacactctccaagtggatgctcaggtcagattatgatgctcttaaataaatgtactgaagcttagaatgtaaagcacacaactatttgcagcagcaatagtctttcaaaataactaaaacaaacttttaaatataaggcatataaaacagactattaaggatagttttccaaactatatatagaaacacaggaaaatatgtgtggcctcataataaagttaaataaatattatttctgagttcttataaacactatgaggttatagttttatttggttcccataaattaaaaactctgattgcttttacataaattcttagctactctcagacttttttttttttgagacggagtctccctctgtcacccaggctggagtgcagcagggcgatctcggctcactgcaacctctgcctgccgggttcaagcaattctcctgcctcagccctgagtagctgggactacaggcacgcaccaccatgccaggctgattttttgtatttttagtagagacagggtttcaccatgctggccaggctggtctcgaactcctggcctcagatgatccgcccaccttggcctcccaaaatgttgggattacaggcgtgagccactgcgcccggccctttcagatttttattaatgtctttttataagacacagagattatctctaacttcatttcagaaatgtgctttttcattggttttaataagtacatttaattttctagcaatgaacatgacttaaaatttaaggttcaaggtagttctagaaaaaggtagacactgaactatctgcttttctacatccccatatttacaaagcctagcatccactgtgctttcctccatacactcaatcacattgtcaataaatagtaactgtggtccaggttacctatgataaagactccaaaattcctcaaaattttacaacactacaaagtcattaatatctgatattgataggttataagtattagtgttatgtaactttttgctattggaaaagaaatacaaatctttatttttgctatctaaattaaaactaagctccatgatcaagataatacctaaaatgtacattcctaaataaaggtaaagctgtttaagggctgaactagtccaatatacaattaagggttatttattcctattcttttgtttttgtttttttgaatccctatgttaaacccgtggtttctcatgaattagatcataatttaacattgtaaaatttcagaaactattgtgctaatatttagatttcaggaaggaatcagactaaatcaattacctccattcattgttagaacagaagatataatagcttactaactgatatgagttatgaatgtcactatgacacaaaatttgctgtgatttgctaatctggctacaagtgcagtatttttcatgaatgtcaacacacagcatttccaacttgtaacatgaaactccagctcataaagagtgtattgtgtgacttgaaaaagtctgattgtaactaagtaacaaccgttcccctgaaaaaacgaacaaaatccattaggaaatcaggcacagacggtattgatcggtttttcttcctttcctcctgtggttttgtttctcaagacatataggtggttccaacagaagccaacacttgttacaaaataacacagctatttttttccttttctttttctttatctttttctcgtggttccttccgtttacgttcactattcccagattgtcttccacttgatggagaggcttgtgctggctggccctgagcctgtgtagaagcagcagcagcagcagctgctgcttgttcctgttcctgatagtattgagaagcccgtctgtcctcttcctcttggagtttctttgctagttccaaatcactgattccttccgggatttgttcccaattgatctcttggctctgctgttcttgttgtagagataatgccataagataatcctgatctatctgatcttgttgtcctttgtatacagtttcaggatctgaaggaggtcgaagatgaaattctgagtcacagaaatttccatcaccatctacgttgtgtaggctttcccaaacaactttctcttcagtaagaaacccctggtccgttaccaacaaatacagttgaccctgagggtctactaaccacccatggtacaaaggaatatcaagaagatcaaatactatgcattctggtgtatattcaaacactcgaacaccagtgaatcttacatttacatccaggcctgtctgtagtttgtgcaaaattgccatggcatcactcatattctgttcataatttaaacgttgaatttctgaaatttcttttggctttgcatcaagcatgtaatctcctaaatattccatcagctgctcagcagttatgatttccatcatcggtggaagtttcaccttccaggccaggagcaaaacattgaggatggccagcaaggggcagggtccgttctcattctgggtgatgatgggtgtgttctcttccttccactggatccacttgatgtgatacacagattgtcccgggaagcgttccttggaggccgccagcacctgagcggtctcctccccctcctcctccttgcacagaggaacagccccgggcaacaccgccgcgccctcctcctcctcagggaccctgttctccgctccctcctcactattgaactcgcagctactgggaaaagaatgcaggttagagaacgactccagagagtccaggctcggagattccccaggagggctcgggtcgctgcaactgctgctgaggccgccggcgctgctgggctcttcggagccggcggcggtcagttctgcttggcaggtgccggcgagatccgggcgggctcccgcgtctccggcggtacccaactcatgacccactccggccacggctgtctccggggaggcggtcaccttgtactgccctctcagaggcgcctcggcggcagcaggactctccaaaccactgtccttcaagtccaaacccgcggaggagctgcagggtccgggaacctcaggagagcccgcgggagaagccgagtccgggaggctcctcctggcggccgccgcccccagcccattcccgccgctggtctccgccgcccataccccaggaccatcaccagcggcgagcctggtctcctgtagcccttcctgcgaagaacctgtccctgacgctggcccggccgccaccccgtgttctagcggctgcaggctctcggggctgctctccataccgggccgcccgcccccagctctatggagaccgcggccacttctccgcagccagcgccttggacgccatgacagctgtattggcagcaacagcgccctggcgcggcctcggtcaggcacgtcaccggggagagtact

SEQ ID NO: 14078 - RNA, 7612 nt, Homo sapiens
  source 1..7612: mol_type = other RNA
gctgggattacaggcatgagccaccgcaccgggccagtttcctgactttttattttcagctataaaacaattatgagagccaaaggagccaggatcaccttccaaaacattttgttttgtccttctctaatttatgaggcattctttcttctcaaagcaggatattacagtgcagattaaaactggatattaaagttaatggtgacaaattattaagtagtttgaagaaatccttagaatatcagataaagagagacttaatggcagaagaagaagtctactggggttcaaagcttaggttttatatttctgccatggtatctcaacactttctctgggatagtacgatgccctaaaaaatacctgtgttaggcagacaagtctaaatctcctttctcaggacaataggacaaaactgaacttgaggcaatagttgaagaattttaccccgtttttcaagtttaattttcttgagatcagaaaagtaaaattagaaagtagaatccttcatgtaaaaaaatatatgcgtatcacaatttattaaactctaacatctaagagcaaaaacaccaggattaagtaagaacatgcatgaactaaaatttagatagatattcaaagtaagttaaatttaccagagtcctgcatctggcctctcccatgccattatcgctattttgcaatttgttttgttcaggaagcctctgattttaatatttaaagtgtcacctgagaagagtaacctcaattcttcatgttttctcaacaatcttagaggtgttggacatcattaataaaatatactaaattatcagagaacttaagaacgctaagattctgatgagttcctttaccattttcagtcactttctaaaagggatttaacttcacattatcaaataacattttacactaaaaacacaatttatatagccctaaaataatattacttgagagatctaaatgaattccaccaatgcaaacgaagtttatatactgtattagtaatttgataccaccgtattccatggagaaaaaggcaaagagaatctaaatatttagatctgtgaaagatactagaaaaaaatagatttttaaatgcttctgatcctctcaaaatactcttgattttgactctatagtctatagaacacacaaaaaactgtaaaatgcatttgggaagagatcacgccatactcaaagaaaattctacaaattttgacagcattaaaaaaactgacttaagatatattttgttattgagaaaaaagtgtgcacattcaagaacataggatgtgtaatatttgtgataaattaagtcatactttgtgcttatactatgccctttattcaggagtgcaaaacacttaatcaaaaagagcatccttcacatatttaaagagtacattgaggcacagaaagtttgcccaaggcaagatagaaagtcgggtttatagacacaaaatgatctagaattcttcatgtccaattccttaaaatacaaactgtagactatttgtaatgcctccatcttattttatcaaacattagtaattttactattataagtttatgcataagtactgtgtgataggtaatgcccataaggtttttatcatgttttaaggtaacttgtgcatggaataggaaaagttaatcaaatgtaatcaattcgcttttgctttttaacaaaacttaaataaatgagctatttgaggacagttctggaaattcttgccttgatttttctccaagattttagatatgtagttcacatgtgaacattaatatatgaacaattattttatttattggcctctagttctctttcctctcatgatctgtctcttagtgaattgactttctgattcattgaaagcaaaatgctaagaaggttttgtgcaagtgcaaaatgtttaatcttgggttcagtcaactagtctctgatactaacttgcttagttaagccaagatcaagaagtatgagaaagaacttgaaatatgataaagaatttgaaacagaatatgggataagtagtcaatatcagaaatgtgagacaataaaaacaagatatattccaaagcctaatcctaaatttaaatctacacttcattcaactctgaacctgaccttgaaacatggaagaagttactttacctaagcacactgcaccagtgtaaaaccaatgccaattttagctgctttatactgcttaatgtgtatatgtacacatgtattcttaaaatggtgattcttaaattgaagttctgaattcttttgagaatctaacagaggtcatgaaaacttgcttcagaaacacacatatgtaaagtacttttaagtgttgatcatgtactataaatcacagcattgtggatgcaatgggattagacatgaagaaaaattttatatttttaataaagactggttactaaccttaaggaatatacttagactctgaaagtaaaaggaaagtgcaatgaccatatttgttcattcatctgcctattttcaaatctaatgatgatttggttgatgcaaatatgtccctaatctaggctataaatgataaaaacaaaaatgtttaagttctaacttttgttagcagtatacatctaagaattttcaagtattacaaaatacttggaaggaaagactttaatataccactttcaaaatcctatgtacccaaaccagcaatgaagtggtgggatatataacgttaccttgggcaaaatttaagaaaataaagacacaatagctctaattttttttttttttttttttttgagacggagtctcgctctattgcccaggcttgcatgcagtggtgctatctcagctcactgcaatcactgcctcctgggttcaagcgattctcctgcctcagcctcccaagtagctgggatgacaggtgcccgccaccatgcctggctaattattgtatttttagtagagacagggttttgccatgttggccaggctggtctcgaactcctgatctcaggtgatccacctgcctcggcctcccaaagtactgggattacaggcatgatctaaattctttatacccttcaagggcaggaaaccagtatctctgaaaagcttgtttgttttaatacaattgaacatttcatctttccccccacagtaatcaaagcaaacattttatcattattattcttggtatatcaaagtaaattccaggaatgtaagaaagtctgacttggaaatattacatagaaaaaggctgaattaacacattacattttttagtttttccttgtaagtatacattgacatctacttatctgatagcagcactgctggttttgagtgagttttgttttgttttgtttccttccagagggaatgcagtatggcagcattttctttggaacaaattaagaagatagtaacaaataacagaagaaatacttctacacatatattttccatgggcaataaacagataagtatataattatgaaaaaatatgcctcaactatgctttttaaaatttctcaaggtatactggtttgtttttcttattcaaatataatgcactatcactactatctgtcccgggaaaaacaaaccctgaggtttgagttacctccttcagccaacagagtgatatcaagagtaaacttggattgaggtcaacctgtttgagccaatagagagttctgtagtatatctggttattttactaacgtatacatattctaggttataatcaagatactcattaaatattttctatcagagttttatatcccaaacaggttctttgatgatttatcatgctaccataggaaatttgaagaaataacaaattgtgtaacagaaatagacatgcaatataaaggacataaaagatacagcttgaccctggatttttcccttagaataattccttccataaataagactctatttttacatacagattcatcctataactggtcttggatcataaagttaatgacatagttgaaaaaatccagaccacacatttttgtggtcttttgtcaccccagaccacacacaaaaaaaacactctccaagtggatgctcaggtcagattatgatgctcttaaataaatgtactgaagcttagaatgtaaagcacacaactatttgcagcagcaatagtctttcaaaataactaaaacaaacttttaaatataaggcatataaaacagactattaaggatagttttccaaactatatatagaaacacaggaaaatatgtgtggcctcataataaagttaaataaatattatttctgagttcttataaacactatgaggttatagttttatttggttcccataaattaaaaactctgattgcttttacataaattcttagctactctcagacttttttttttttgagacggagtctccctctgtcacccaggctggagtgcagcagggcgatctcggctcactgcaacctctgcctgccgggttcaagcaattctcctgcctcagccctgagtagctgggactacaggcacgcaccaccatgccaggctgattttttgtatttttagtagagacagggtttcaccatgctggccaggctggtctcgaactcctggcctcagatgatccgcccaccttggcctcccaaaatgttgggattacaggcgtgagccactgcgcccggccctttcagatttttattaatgtctttttataagacacagagattatctctaacttcatttcagaaatgtgctttttcattggttttaataagtacatttaattttctagcaatgaacatgacttaaaatttaaggttcaaggtagttctagaaaaaggtagacactgaactatctgcttttctacatccccatatttacaaagcctagcatccactgtgctttcctccatacactcaatcacattgtcaataaatagtaactgtggtccaggttacctatgataaagactccaaaattcctcaaaattttacaacactacaaagtcattaatatctgatattgataggttataagtattagtgttatgtaactttttgctattggaaaagaaatacaaatctttatttttgctatctaaattaaaactaagctccatgatcaagataatacctaaaatgtacattcctaaataaaggtaaagctgtttaagggctgaactagtccaatatacaattaagggttatttattcctattcttttgtttttgtttttttgaatccctatgttaaacccgtggtttctcatgaattagatcataatttaacattgtaaaatttcagaaactattgtgctaatatttagatttcaggaaggaatcagactaaatcaattacctccattcattgttagaacagaagatataatagcttactaactgatatgagttatgaatgtcactatgacacaaaatttgctgtgatttgctaatctggctacaagtgcagtatttttcatgaatgtcaacacacagcatttccaacttgtaacatgaaactccagctcataaagagtgtattgtgtgacttgaaaaagtctgattgtaactaagtaacaaccgttcccctgaaaaaacgaacaaaatccattaggaaatcaggcacagacggtattgatcggtttttcttcctttcctcctgtggttttgtttctcaagacatataggtggttccaacagaagccaacacttgttacaaaataacacagctatttttttccttttctttttctttatctttttctcgtggttccttccgtttacgttcactattcccagattgtcttccacttgatggagaggcttgtgctggctggccctgagcctgtgtagaagcagcagcagcagcagctgctgcttgttcctgttcctgatagtattgagaagcccgtctgtcctcttcctcttggagtttctttgctagttccaaatcactgattccttccgggatttgttcccaattgatctcttggctctgctgttcttgttgtagagataatgccataagataatcctgatctatctgatcttgttgtcctttgtatacagtttcaggatctgaaggaggtcgaagatgaaattctgagtcacagaaatttccatcaccatctacgttgtgtaggctttcccaaacaactttctcttcagtaagaaacccctggtccgttaccaacaaatacagttgacccttgtatttggtcatggtgctaaaatgattattccgaaagaacacacaaagttctccttcctgaaccgttgaagttagttcacataatccatggtatgtcagttgagtggctgtgttatttagaaactgctcagctacaaagccttcactaaccagctcactattgtctgactgtttacaagagatgatcttctccactagttggttgtagctgcagttaccaacagcttttacaatgtcatcaatatttacatccaggcctgtctgtagtttgtgcaaaattgccatggcatcactcatattctgttcataatttaaacgttgaatttctgaaatttcttttggctttgcatcaagcatgtaatctcctaaatattccatcagctgctcagcagttatgatttccatcatcggtggaagtttcaccttccaggccaggagcaaaacattgaggatggccagcaaggggcagggtccgttctcattctgggtgatgatgggtgtgttctcttccttccactggatccacttgatgtgatacacagattgtcccgggaagcgttccttggaggccgccagcacctgagcggtctcctccccctcctcctccttgcacagaggaacagccccgggcaacaccgccgcgccctcctcctcctcagggaccctgttctccgctccctcctcactattgaactcgcagctactgggaaaagaatgcaggttagagaacgactccagagagtccaggctcggagattccccaggagggctcgggtcgctgcaactgctgctgaggccgccggcgctgctgggctcttcggagccggcggcggtcagttctgcttggcaggtgccggcgagatccgggcgggctcccgcgtctccggcggtacccaactcatgacccactccggccacggctgtctccggggaggcggtcaccttgtactgccctctcagaggcgcctcggcggcagcaggactctccaaaccactgtccttcaagtccaaacccgcggaggagctgcagggtccgggaacctcaggagagcccgcgggagaagccgagtccgggaggctcctcctggcggccgccgcccccagcccattcccgccgctggtctccgccgcccataccccaggaccatcaccagcggcgagcctggtctcctgtagcccttcctgcgaagaacctgtccctgacgctggcccggccgccaccccgtgttctagcggctgcaggctctcggggctgctctccataccgggccgcccgcccccagctctatggagaccgcggccacttctccgcagccagcgccttggacgccatgacagctgtattggcagcaacagcgccctggcgcggcctcggtcaggcacgtcaccggggagagtact

SEQ ID NO: 14079 - RNA, 7768 nt, Homo sapiens
  source 1..7768: mol_type = other RNA
gctgggattacaggcatgagccaccgcaccgggccagtttcctgactttttattttcagctataaaacaattatgagagccaaaggagccaggatcaccttccaaaacattttgttttgtccttctctaatttatgaggcattctttcttctcaaagcaggatattacagtgcagattaaaactggatattaaagttaatggtgacaaattattaagtagtttgaagaaatccttagaatatcagataaagagagacttaatggcagaagaagaagtctactggggttcaaagcttaggttttatatttctgccatggtatctcaacactttctctgggatagtacgatgccctaaaaaatacctgtgttaggcagacaagtctaaatctcctttctcaggacaataggacaaaactgaacttgaggcaatagttgaagaattttaccccgtttttcaagtttaattttcttgagatcagaaaagtaaaattagaaagtagaatccttcatgtaaaaaaatatatgcgtatcacaatttattaaactctaacatctaagagcaaaaacaccaggattaagtaagaacatgcatgaactaaaatttagatagatattcaaagtaagttaaatttaccagagtcctgcatctggcctctcccatgccattatcgctattttgcaatttgttttgttcaggaagcctctgattttaatatttaaagtgtcacctgagaagagtaacctcaattcttcatgttttctcaacaatcttagaggtgttggacatcattaataaaatatactaaattatcagagaacttaagaacgctaagattctgatgagttcctttaccattttcagtcactttctaaaagggatttaacttcacattatcaaataacattttacactaaaaacacaatttatatagccctaaaataatattacttgagagatctaaatgaattccaccaatgcaaacgaagtttatatactgtattagtaatttgataccaccgtattccatggagaaaaaggcaaagagaatctaaatatttagatctgtgaaagatactagaaaaaaatagatttttaaatgcttctgatcctctcaaaatactcttgattttgactctatagtctatagaacacacaaaaaactgtaaaatgcatttgggaagagatcacgccatactcaaagaaaattctacaaattttgacagcattaaaaaaactgacttaagatatattttgttattgagaaaaaagtgtgcacattcaagaacataggatgtgtaatatttgtgataaattaagtcatactttgtgcttatactatgccctttattcaggagtgcaaaacacttaatcaaaaagagcatccttcacatatttaaagagtacattgaggcacagaaagtttgcccaaggcaagatagaaagtcgggtttatagacacaaaatgatctagaattcttcatgtccaattccttaaaatacaaactgtagactatttgtaatgcctccatcttattttatcaaacattagtaattttactattataagtttatgcataagtactgtgtgataggtaatgcccataaggtttttatcatgttttaaggtaacttgtgcatggaataggaaaagttaatcaaatgtaatcaattcgcttttgctttttaacaaaacttaaataaatgagctatttgaggacagttctggaaattcttgccttgatttttctccaagattttagatatgtagttcacatgtgaacattaatatatgaacaattattttatttattggcctctagttctctttcctctcatgatctgtctcttagtgaattgactttctgattcattgaaagcaaaatgctaagaaggttttgtgcaagtgcaaaatgtttaatcttgggttcagtcaactagtctctgatactaacttgcttagttaagccaagatcaagaagtatgagaaagaacttgaaatatgataaagaatttgaaacagaatatgggataagtagtcaatatcagaaatgtgagacaataaaaacaagatatattccaaagcctaatcctaaatttaaatctacacttcattcaactctgaacctgaccttgaaacatggaagaagttactttacctaagcacactgcaccagtgtaaaaccaatgccaattttagctgctttatactgcttaatgtgtatatgtacacatgtattcttaaaatggtgattcttaaattgaagttctgaattcttttgagaatctaacagaggtcatgaaaacttgcttcagaaacacacatatgtaaagtacttttaagtgttgatcatgtactataaatcacagcattgtggatgcaatgggattagacatgaagaaaaattttatatttttaataaagactggttactaaccttaaggaatatacttagactctgaaagtaaaaggaaagtgcaatgaccatatttgttcattcatctgcctattttcaaatctaatgatgatttggttgatgcaaatatgtccctaatctaggctataaatgataaaaacaaaaatgtttaagttctaacttttgttagcagtatacatctaagaattttcaagtattacaaaatacttggaaggaaagactttaatataccactttcaaaatcctatgtacccaaaccagcaatgaagtggtgggatatataacgttaccttgggcaaaatttaagaaaataaagacacaatagctctaattttttttttttttttttttttgagacggagtctcgctctattgcccaggcttgcatgcagtggtgctatctcagctcactgcaatcactgcctcctgggttcaagcgattctcctgcctcagcctcccaagtagctgggatgacaggtgcccgccaccatgcctggctaattattgtatttttagtagagacagggttttgccatgttggccaggctggtctcgaactcctgatctcaggtgatccacctgcctcggcctcccaaagtactgggattacaggcatgatctaaattctttatacccttcaagggcaggaaaccagtatctctgaaaagcttgtttgttttaatacaattgaacatttcatctttccccccacagtaatcaaagcaaacattttatcattattattcttggtatatcaaagtaaattccaggaatgtaagaaagtctgacttggaaatattacatagaaaaaggctgaattaacacattacattttttagtttttccttgtaagtatacattgacatctacttatctgatagcagcactgctggttttgagtgagttttgttttgttttgtttccttccagagggaatgcagtatggcagcattttctttggaacaaattaagaagatagtaacaaataacagaagaaatacttctacacatatattttccatgggcaataaacagataagtatataattatgaaaaaatatgcctcaactatgctttttaaaatttctcaaggtatactggtttgtttttcttattcaaatataatgcactatcactactatctgtcccgggaaaaacaaaccctgaggtttgagttacctccttcagccaacagagtgatatcaagagtaaacttggattgaggtcaacctgtttgagccaatagagagttctgtagtatatctggttattttactaacgtatacatattctaggttataatcaagatactcattaaatattttctatcagagttttatatcccaaacaggttctttgatgatttatcatgctaccataggaaatttgaagaaataacaaattgtgtaacagaaatagacatgcaatataaaggacataaaagatacagcttgaccctggatttttcccttagaataattccttccataaataagactctatttttacatacagattcatcctataactggtcttggatcataaagttaatgacatagttgaaaaaatccagaccacacatttttgtggtcttttgtcaccccagaccacacacaaaaaaaacactctccaagtggatgctcaggtcagattatgatgctcttaaataaatgtactgaagcttagaatgtaaagcacacaactatttgcagcagcaatagtctttcaaaataactaaaacaaacttttaaatataaggcatataaaacagactattaaggatagttttccaaactatatatagaaacacaggaaaatatgtgtggcctcataataaagttaaataaatattatttctgagttcttataaacactatgaggttatagttttatttggttcccataaattaaaaactctgattgcttttacataaattcttagctactctcagacttttttttttttgagacggagtctccctctgtcacccaggctggagtgcagcagggcgatctcggctcactgcaacctctgcctgccgggttcaagcaattctcctgcctcagccctgagtagctgggactacaggcacgcaccaccatgccaggctgattttttgtatttttagtagagacagggtttcaccatgctggccaggctggtctcgaactcctggcctcagatgatccgcccaccttggcctcccaaaatgttgggattacaggcgtgagccactgcgcccggccctttcagatttttattaatgtctttttataagacacagagattatctctaacttcatttcagaaatgtgctttttcattggttttaataagtacatttaattttctagcaatgaacatgacttaaaatttaaggttcaaggtagttctagaaaaaggtagacactgaactatctgcttttctacatccccatatttacaaagcctagcatccactgtgctttcctccatacactcaatcacattgtcaataaatagtaactgtggtccaggttacctatgataaagactccaaaattcctcaaaattttacaacactacaaagtcattaatatctgatattgataggttataagtattagtgttatgtaactttttgctattggaaaagaaatacaaatctttatttttgctatctaaattaaaactaagctccatgatcaagataatacctaaaatgtacattcctaaataaaggtaaagctgtttaagggctgaactagtccaatatacaattaagggttatttattcctattcttttgtttttgtttttttgaatccctatgttaaacccgtggtttctcatgaattagatcataatttaacattgtaaaatttcagaaactattgtgctaatatttagatttcaggaaggaatcagactaaatcaattacctccattcattgttagaacagaagatataatagcttactaactgatatgagttatgaatgtcactatgacacaaaatttgctgtgatttgctaatctggctacaagtgcagtatttttcatgaatgtcaacacacagcatttccaacttgtaacatgaaactccagctcataaagagtgtattgtgtgacttgaaaaagtctgattgtaactaagtaacaaccgttcccctgaaaaaacgaacaaaatccattaggaaatcaggcacagacggtattgatcggtttttcttcctttcctcctgtggttttgtttctcaagacatataggtggttccaacagaagccaacacttgttacaaaataacacagctatttttttccttttctttttctttatctttttctcgtggttccttccgtttacgttcactattcccagattgtcttccacttgatggagaggcttgtgctggctggccctgagcctgtgtagaagcagcagcagcagcagctgctgcttgttcctgttcctgatagtattgagaagcccgtctgtcctcttcctcttggagtttctttgctagttccaaatcactgattccttccgggatttgttcccaattgatctcttggctctgctgttcttgttgtagagataatgccataagataatcctgatctatctgatcttgttgtcctttgtatacagtttcaggatctgaaggaggtcgaagatgaaattctgagtcacagaaatttccatcaccatctacgttgtgtaggctttcccaaacaactttctcttcagtaagaaacccctggtccgttaccaacaaatacagttgacccttgtatttggtcatggtgctaaaatgattattccgaaagaacacacaaagttctccttcctgaaccgttgaagttagttcacataatccatggtatgtcagttgagtggctgtgttatttagaaactgctcagctacaaagccttcactaaccagctcactattgtctgactgtttacaagagatgatcttctccactagttggttgtagctgcagttaccaacagcttttacaatgtcatcaatctgagggtctactaaccacccatggtacaaaggaatatcaagaagatcaaatactatgcattctggtgtatattcaaacactcgaacaccagtgaatcttacatttacatccaggcctgtctgtagtttgtgcaaaattgccatggcatcactcatattattttttcccttaagtgttttagaacttttcttaaatctacagcaatgatgaatctgttcataatttaaacgttgaatttctgaaatttcttttggctttgcatcaagcatgtaatctcctaaatattccatcagctgctcagcagttatgatttccatcatcggtggaagtttcaccttccaggccaggagcaaaacattgaggatggccagcaaggggcagggtccgttctcattctgggtgatgatgggtgtgttctcttccttccactggatccacttgatgtgatacacagattgtcccgggaagcgttccttggaggccgccagcacctgagcggtctcctccccctcctcctccttgcacagaggaacagccccgggcaacaccgccgcgccctcctcctcctcagggaccctgttctccgctccctcctcactattgaactcgcagctactgggaaaagaatgcaggttagagaacgactccagagagtccaggctcggagattccccaggagggctcgggtcgctgcaactgctgctgaggccgccggcgctgctgggctcttcggagccggcggcggtcagttctgcttggcaggtgccggcgagatccgggcgggctcccgcgtctccggcggtacccaactcatgacccactccggccacggctgtctccggggaggcggtcaccttgtactgccctctcagaggcgcctcggcggcagcaggactctccaaaccactgtccttcaagtccaaacccgcggaggagctgcagggtccgggaacctcaggagagcccgcgggagaagccgagtccgggaggctcctcctggcggccgccgcccccagcccattcccgccgctggtctccgccgcccataccccaggaccatcaccagcggcgagcctggtctcctgtagcccttcctgcgaagaacctgtccctgacgctggcccggccgccaccccgtgttctagcggctgcaggctctcggggctgctctccataccgggccgcccgcccccagctctatggagaccgcggccacttctccgcagccagcgccttggacgccatgacagctgtattggcagcaacagcgccctggcgcggcctcggtcaggcacgtcaccggggagagtact

SEQ ID NO: 14080 - RNA, 7670 nt, Homo sapiens
  source 1..7670: mol_type = other RNA
gctgggattacaggcatgagccaccgcaccgggccagtttcctgactttttattttcagctataaaacaattatgagagccaaaggagccaggatcaccttccaaaacattttgttttgtccttctctaatttatgaggcattctttcttctcaaagcaggatattacagtgcagattaaaactggatattaaagttaatggtgacaaattattaagtagtttgaagaaatccttagaatatcagataaagagagacttaatggcagaagaagaagtctactggggttcaaagcttaggttttatatttctgccatggtatctcaacactttctctgggatagtacgatgccctaaaaaatacctgtgttaggcagacaagtctaaatctcctttctcaggacaataggacaaaactgaacttgaggcaatagttgaagaattttaccccgtttttcaagtttaattttcttgagatcagaaaagtaaaattagaaagtagaatccttcatgtaaaaaaatatatgcgtatcacaatttattaaactctaacatctaagagcaaaaacaccaggattaagtaagaacatgcatgaactaaaatttagatagatattcaaagtaagttaaatttaccagagtcctgcatctggcctctcccatgccattatcgctattttgcaatttgttttgttcaggaagcctctgattttaatatttaaagtgtcacctgagaagagtaacctcaattcttcatgttttctcaacaatcttagaggtgttggacatcattaataaaatatactaaattatcagagaacttaagaacgctaagattctgatgagttcctttaccattttcagtcactttctaaaagggatttaacttcacattatcaaataacattttacactaaaaacacaatttatatagccctaaaataatattacttgagagatctaaatgaattccaccaatgcaaacgaagtttatatactgtattagtaatttgataccaccgtattccatggagaaaaaggcaaagagaatctaaatatttagatctgtgaaagatactagaaaaaaatagatttttaaatgcttctgatcctctcaaaatactcttgattttgactctatagtctatagaacacacaaaaaactgtaaaatgcatttgggaagagatcacgccatactcaaagaaaattctacaaattttgacagcattaaaaaaactgacttaagatatattttgttattgagaaaaaagtgtgcacattcaagaacataggatgtgtaatatttgtgataaattaagtcatactttgtgcttatactatgccctttattcaggagtgcaaaacacttaatcaaaaagagcatccttcacatatttaaagagtacattgaggcacagaaagtttgcccaaggcaagatagaaagtcgggtttatagacacaaaatgatctagaattcttcatgtccaattccttaaaatacaaactgtagactatttgtaatgcctccatcttattttatcaaacattagtaattttactattataagtttatgcataagtactgtgtgataggtaatgcccataaggtttttatcatgttttaaggtaacttgtgcatggaataggaaaagttaatcaaatgtaatcaattcgcttttgctttttaacaaaacttaaataaatgagctatttgaggacagttctggaaattcttgccttgatttttctccaagattttagatatgtagttcacatgtgaacattaatatatgaacaattattttatttattggcctctagttctctttcctctcatgatctgtctcttagtgaattgactttctgattcattgaaagcaaaatgctaagaaggttttgtgcaagtgcaaaatgtttaatcttgggttcagtcaactagtctctgatactaacttgcttagttaagccaagatcaagaagtatgagaaagaacttgaaatatgataaagaatttgaaacagaatatgggataagtagtcaatatcagaaatgtgagacaataaaaacaagatatattccaaagcctaatcctaaatttaaatctacacttcattcaactctgaacctgaccttgaaacatggaagaagttactttacctaagcacactgcaccagtgtaaaaccaatgccaattttagctgctttatactgcttaatgtgtatatgtacacatgtattcttaaaatggtgattcttaaattgaagttctgaattcttttgagaatctaacagaggtcatgaaaacttgcttcagaaacacacatatgtaaagtacttttaagtgttgatcatgtactataaatcacagcattgtggatgcaatgggattagacatgaagaaaaattttatatttttaataaagactggttactaaccttaaggaatatacttagactctgaaagtaaaaggaaagtgcaatgaccatatttgttcattcatctgcctattttcaaatctaatgatgatttggttgatgcaaatatgtccctaatctaggctataaatgataaaaacaaaaatgtttaagttctaacttttgttagcagtatacatctaagaattttcaagtattacaaaatacttggaaggaaagactttaatataccactttcaaaatcctatgtacccaaaccagcaatgaagtggtgggatatataacgttaccttgggcaaaatttaagaaaataaagacacaatagctctaattttttttttttttttttttttgagacggagtctcgctctattgcccaggcttgcatgcagtggtgctatctcagctcactgcaatcactgcctcctgggttcaagcgattctcctgcctcagcctcccaagtagctgggatgacaggtgcccgccaccatgcctggctaattattgtatttttagtagagacagggttttgccatgttggccaggctggtctcgaactcctgatctcaggtgatccacctgcctcggcctcccaaagtactgggattacaggcatgatctaaattctttatacccttcaagggcaggaaaccagtatctctgaaaagcttgtttgttttaatacaattgaacatttcatctttccccccacagtaatcaaagcaaacattttatcattattattcttggtatatcaaagtaaattccaggaatgtaagaaagtctgacttggaaatattacatagaaaaaggctgaattaacacattacattttttagtttttccttgtaagtatacattgacatctacttatctgatagcagcactgctggttttgagtgagttttgttttgttttgtttccttccagagggaatgcagtatggcagcattttctttggaacaaattaagaagatagtaacaaataacagaagaaatacttctacacatatattttccatgggcaataaacagataagtatataattatgaaaaaatatgcctcaactatgctttttaaaatttctcaaggtatactggtttgtttttcttattcaaatataatgcactatcactactatctgtcccgggaaaaacaaaccctgaggtttgagttacctccttcagccaacagagtgatatcaagagtaaacttggattgaggtcaacctgtttgagccaatagagagttctgtagtatatctggttattttactaacgtatacatattctaggttataatcaagatactcattaaatattttctatcagagttttatatcccaaacaggttctttgatgatttatcatgctaccataggaaatttgaagaaataacaaattgtgtaacagaaatagacatgcaatataaaggacataaaagatacagcttgaccctggatttttcccttagaataattccttccataaataagactctatttttacatacagattcatcctataactggtcttggatcataaagttaatgacatagttgaaaaaatccagaccacacatttttgtggtcttttgtcaccccagaccacacacaaaaaaaacactctccaagtggatgctcaggtcagattatgatgctcttaaataaatgtactgaagcttagaatgtaaagcacacaactatttgcagcagcaatagtctttcaaaataactaaaacaaacttttaaatataaggcatataaaacagactattaaggatagttttccaaactatatatagaaacacaggaaaatatgtgtggcctcataataaagttaaataaatattatttctgagttcttataaacactatgaggttatagttttatttggttcccataaattaaaaactctgattgcttttacataaattcttagctactctcagacttttttttttttgagacggagtctccctctgtcacccaggctggagtgcagcagggcgatctcggctcactgcaacctctgcctgccgggttcaagcaattctcctgcctcagccctgagtagctgggactacaggcacgcaccaccatgccaggctgattttttgtatttttagtagagacagggtttcaccatgctggccaggctggtctcgaactcctggcctcagatgatccgcccaccttggcctcccaaaatgttgggattacaggcgtgagccactgcgcccggccctttcagatttttattaatgtctttttataagacacagagattatctctaacttcatttcagaaatgtgctttttcattggttttaataagtacatttaattttctagcaatgaacatgacttaaaatttaaggttcaaggtagttctagaaaaaggtagacactgaactatctgcttttctacatccccatatttacaaagcctagcatccactgtgctttcctccatacactcaatcacattgtcaataaatagtaactgtggtccaggttacctatgataaagactccaaaattcctcaaaattttacaacactacaaagtcattaatatctgatattgataggttataagtattagtgttatgtaactttttgctattggaaaagaaatacaaatctttatttttgctatctaaattaaaactaagctccatgatcaagataatacctaaaatgtacattcctaaataaaggtaaagctgtttaagggctgaactagtccaatatacaattaagggttatttattcctattcttttgtttttgtttttttgaatccctatgttaaacccgtggtttctcatgaattagatcataatttaacattgtaaaatttcagaaactattgtgctaatatttagatttcaggaaggaatcagactaaatcaattacctccattcattgttagaacagaagatataatagcttactaactgatatgagttatgaatgtcactatgacacaaaatttgctgtgatttgctaatctggctacaagtgcagtatttttcatgaatgtcaacacacagcatttccaacttgtaacatgaaactccagctcataaagagtgtattgtgtgacttgaaaaagtctgattgtaactaagtaacaaccgttcccctgaaaaaacgaacaaaatccattaggaaatcaggcacagacggtattgatcggtttttcttcctttcctcctgtggttttgtttctcaagacatataggtggttccaacagaagccaacacttgttacaaaataacacagctatttttttccttttctttttctttatctttttctcgtggttccttccgtttacgttcactattcccagattgtcttccacttgatggagaggcttgtgctggctggccctgagcctgtgtagaagcagcagcagcagcagctgctgcttgttcctgttcctgatagtattgagaagcccgtctgtcctcttcctcttggagtttctttgctagttccaaatcactgattccttccgggatttgttcccaattgatctcttggctctgctgttcttgttgtagagataatgccataagataatcctgatctatctgatcttgttgtcctttgtatacagtttcaggatctgaaggaggtcgaagatgaaattctgagtcacagaaatttccatcaccatctacgttgtgtaggctttcccaaacaactttctcttcagtaagaaacccctggtccgttaccaacaaatacagttgacccttgtatttggtcatggtgctaaaatgattattccgaaagaacacacaaagttctccttcctgaaccgttgaagttagttcacataatccatggtatgtcagttgagtggctgtgttatttagaaactgctcagctacaaagccttcactaaccagctcactattgtctgactgtttacaagagatgatcttctccactagttggttgtagctgcagttaccaacagcttttacaatgtcatcaatctgagggtctactaaccacccatggtacaaaggaatatcaagaagatcaaatactatgcattctggtgtatattcaaacactcgaacaccagtgaatcttacatttacatccaggcctgtctgtagtttgtgcaaaattgccatggcatcactcatattctgttcataatttaaacgttgaatttctgaaatttcttttggctttgcatcaagcatgtaatctcctaaatattccatcagctgctcagcagttatgatttccatcatcggtggaagtttcaccttccaggccaggagcaaaacattgaggatggccagcaaggggcagggtccgttctcattctgggtgatgatgggtgtgttctcttccttccactggatccacttgatgtgatacacagattgtcccgggaagcgttccttggaggccgccagcacctgagcggtctcctccccctcctcctccttgcacagaggaacagccccgggcaacaccgccgcgccctcctcctcctcagggaccctgttctccgctccctcctcactattgaactcgcagctactgggaaaagaatgcaggttagagaacgactccagagagtccaggctcggagattccccaggagggctcgggtcgctgcaactgctgctgaggccgccggcgctgctgggctcttcggagccggcggcggtcagttctgcttggcaggtgccggcgagatccgggcgggctcccgcgtctccggcggtacccaactcatgacccactccggccacggctgtctccggggaggcggtcaccttgtactgccctctcagaggcgcctcggcggcagcaggactctccaaaccactgtccttcaagtccaaacccgcggaggagctgcagggtccgggaacctcaggagagcccgcgggagaagccgagtccgggaggctcctcctggcggccgccgcccccagcccattcccgccgctggtctccgccgcccataccccaggaccatcaccagcggcgagcctggtctcctgtagcccttcctgcgaagaacctgtccctgacgctggcccggccgccaccccgtgttctagcggctgcaggctctcggggctgctctccataccgggccgcccgcccccagctctatggagaccgcggccacttctccgcagccagcgccttggacgccatgacagctgtattggcagcaacagc

SEQ ID NO: 14081 - RNA, 7525 nt, Homo sapiens
  source 1..7525: mol_type = other RNA
gctgggattacaggcatgagccaccgcaccgggccagtttcctgactttttattttcagctataaaacaattatgagagccaaaggagccaggatcaccttccaaaacattttgttttgtccttctctaatttatgaggcattctttcttctcaaagcaggatattacagtgcagattaaaactggatattaaagttaatggtgacaaattattaagtagtttgaagaaatccttagaatatcagataaagagagacttaatggcagaagaagaagtctactggggttcaaagcttaggttttatatttctgccatggtatctcaacactttctctgggatagtacgatgccctaaaaaatacctgtgttaggcagacaagtctaaatctcctttctcaggacaataggacaaaactgaacttgaggcaatagttgaagaattttaccccgtttttcaagtttaattttcttgagatcagaaaagtaaaattagaaagtagaatccttcatgtaaaaaaatatatgcgtatcacaatttattaaactctaacatctaagagcaaaaacaccaggattaagtaagaacatgcatgaactaaaatttagatagatattcaaagtaagttaaatttaccagagtcctgcatctggcctctcccatgccattatcgctattttgcaatttgttttgttcaggaagcctctgattttaatatttaaagtgtcacctgagaagagtaacctcaattcttcatgttttctcaacaatcttagaggtgttggacatcattaataaaatatactaaattatcagagaacttaagaacgctaagattctgatgagttcctttaccattttcagtcactttctaaaagggatttaacttcacattatcaaataacattttacactaaaaacacaatttatatagccctaaaataatattacttgagagatctaaatgaattccaccaatgcaaacgaagtttatatactgtattagtaatttgataccaccgtattccatggagaaaaaggcaaagagaatctaaatatttagatctgtgaaagatactagaaaaaaatagatttttaaatgcttctgatcctctcaaaatactcttgattttgactctatagtctatagaacacacaaaaaactgtaaaatgcatttgggaagagatcacgccatactcaaagaaaattctacaaattttgacagcattaaaaaaactgacttaagatatattttgttattgagaaaaaagtgtgcacattcaagaacataggatgtgtaatatttgtgataaattaagtcatactttgtgcttatactatgccctttattcaggagtgcaaaacacttaatcaaaaagagcatccttcacatatttaaagagtacattgaggcacagaaagtttgcccaaggcaagatagaaagtcgggtttatagacacaaaatgatctagaattcttcatgtccaattccttaaaatacaaactgtagactatttgtaatgcctccatcttattttatcaaacattagtaattttactattataagtttatgcataagtactgtgtgataggtaatgcccataaggtttttatcatgttttaaggtaacttgtgcatggaataggaaaagttaatcaaatgtaatcaattcgcttttgctttttaacaaaacttaaataaatgagctatttgaggacagttctggaaattcttgccttgatttttctccaagattttagatatgtagttcacatgtgaacattaatatatgaacaattattttatttattggcctctagttctctttcctctcatgatctgtctcttagtgaattgactttctgattcattgaaagcaaaatgctaagaaggttttgtgcaagtgcaaaatgtttaatcttgggttcagtcaactagtctctgatactaacttgcttagttaagccaagatcaagaagtatgagaaagaacttgaaatatgataaagaatttgaaacagaatatgggataagtagtcaatatcagaaatgtgagacaataaaaacaagatatattccaaagcctaatcctaaatttaaatctacacttcattcaactctgaacctgaccttgaaacatggaagaagttactttacctaagcacactgcaccagtgtaaaaccaatgccaattttagctgctttatactgcttaatgtgtatatgtacacatgtattcttaaaatggtgattcttaaattgaagttctgaattcttttgagaatctaacagaggtcatgaaaacttgcttcagaaacacacatatgtaaagtacttttaagtgttgatcatgtactataaatcacagcattgtggatgcaatgggattagacatgaagaaaaattttatatttttaataaagactggttactaaccttaaggaatatacttagactctgaaagtaaaaggaaagtgcaatgaccatatttgttcattcatctgcctattttcaaatctaatgatgatttggttgatgcaaatatgtccctaatctaggctataaatgataaaaacaaaaatgtttaagttctaacttttgttagcagtatacatctaagaattttcaagtattacaaaatacttggaaggaaagactttaatataccactttcaaaatcctatgtacccaaaccagcaatgaagtggtgggatatataacgttaccttgggcaaaatttaagaaaataaagacacaatagctctaattttttttttttttttttttttgagacggagtctcgctctattgcccaggcttgcatgcagtggtgctatctcagctcactgcaatcactgcctcctgggttcaagcgattctcctgcctcagcctcccaagtagctgggatgacaggtgcccgccaccatgcctggctaattattgtatttttagtagagacagggttttgccatgttggccaggctggtctcgaactcctgatctcaggtgatccacctgcctcggcctcccaaagtactgggattacaggcatgatctaaattctttatacccttcaagggcaggaaaccagtatctctgaaaagcttgtttgttttaatacaattgaacatttcatctttccccccacagtaatcaaagcaaacattttatcattattattcttggtatatcaaagtaaattccaggaatgtaagaaagtctgacttggaaatattacatagaaaaaggctgaattaacacattacattttttagtttttccttgtaagtatacattgacatctacttatctgatagcagcactgctggttttgagtgagttttgttttgttttgtttccttccagagggaatgcagtatggcagcattttctttggaacaaattaagaagatagtaacaaataacagaagaaatacttctacacatatattttccatgggcaataaacagataagtatataattatgaaaaaatatgcctcaactatgctttttaaaatttctcaaggtatactggtttgtttttcttattcaaatataatgcactatcactactatctgtcccgggaaaaacaaaccctgaggtttgagttacctccttcagccaacagagtgatatcaagagtaaacttggattgaggtcaacctgtttgagccaatagagagttctgtagtatatctggttattttactaacgtatacatattctaggttataatcaagatactcattaaatattttctatcagagttttatatcccaaacaggttctttgatgatttatcatgctaccataggaaatttgaagaaataacaaattgtgtaacagaaatagacatgcaatataaaggacataaaagatacagcttgaccctggatttttcccttagaataattccttccataaataagactctatttttacatacagattcatcctataactggtcttggatcataaagttaatgacatagttgaaaaaatccagaccacacatttttgtggtcttttgtcaccccagaccacacacaaaaaaaacactctccaagtggatgctcaggtcagattatgatgctcttaaataaatgtactgaagcttagaatgtaaagcacacaactatttgcagcagcaatagtctttcaaaataactaaaacaaacttttaaatataaggcatataaaacagactattaaggatagttttccaaactatatatagaaacacaggaaaatatgtgtggcctcataataaagttaaataaatattatttctgagttcttataaacactatgaggttatagttttatttggttcccataaattaaaaactctgattgcttttacataaattcttagctactctcagacttttttttttttgagacggagtctccctctgtcacccaggctggagtgcagcagggcgatctcggctcactgcaacctctgcctgccgggttcaagcaattctcctgcctcagccctgagtagctgggactacaggcacgcaccaccatgccaggctgattttttgtatttttagtagagacagggtttcaccatgctggccaggctggtctcgaactcctggcctcagatgatccgcccaccttggcctcccaaaatgttgggattacaggcgtgagccactgcgcccggccctttcagatttttattaatgtctttttataagacacagagattatctctaacttcatttcagaaatgtgctttttcattggttttaataagtacatttaattttctagcaatgaacatgacttaaaatttaaggttcaaggtagttctagaaaaaggtagacactgaactatctgcttttctacatccccatatttacaaagcctagcatccactgtgctttcctccatacactcaatcacattgtcaataaatagtaactgtggtccaggttacctatgataaagactccaaaattcctcaaaattttacaacactacaaagtcattaatatctgatattgataggttataagtattagtgttatgtaactttttgctattggaaaagaaatacaaatctttatttttgctatctaaattaaaactaagctccatgatcaagataatacctaaaatgtacattcctaaataaaggtaaagctgtttaagggctgaactagtccaatatacaattaagggttatttattcctattcttttgtttttgtttttttgaatccctatgttaaacccgtggtttctcatgaattagatcataatttaacattgtaaaatttcagaaactattgtgctaatatttagatttcaggaaggaatcagactaaatcaattacctccattcattgttagaacagaagatataatagcttactaactgatatgagttatgaatgtcactatgacacaaaatttgctgtgatttgctaatctggctacaagtgcagtatttttcatgaatgtcaacacacagcatttccaacttgtaacatgaaactccagctcataaagagtgtattgtgtgacttgaaaaagtctgattgtaactaagtaacaaccgttcccctgaaaaaacgaacaaaatccattaggaaatcaggcacagacggtattgatcggtttttcttcctttcctcctgtggttttgtttctcaagacatataggtggttccaacagaagccaacacttgttacaaaataacacagctatttttttccttttctttttctttatctttttctcgtggttccttccgtttacgttcactattcccagattgtcttccacttgatggagaggcttgtgctggctggccctgctgagcctgtgtagaagcagcagcagcagcagctgctgcttgttcctgttcctgatagtattgagaagcccgtctgtcctcttcctcttggagtttctttgctagttccaaatcactgattccttccgggatttgttcccaattgatctcttggctctgctgttcttgttgtagagataatgccataagataatcctgatctatctgatcttgttgtcctttgtatacagtttcaggatctgaaggaggtcgaagatgaaattctgagtcacagaaatttccatcaccatctacgttgtgtaggctttcccaaacaactttctcttcagtaagaaacccctggtccgttaccaacaaatacagttgaccctgagggtctactaaccacccatggtacaaaggaatatcaagaagatcaaatactatgcattctggtgtatattcaaacactcgaacaccagtgaatcttacatttacatccaggcctgtctgtagtttgtgcaaaattgccatggcatcactcatattattttttcccttaagtgttttagaacttttcttaaatctacagcaatgatgaatctgttcataatttaaacgttgaatttctgaaatttcttttggctttgcatcaagcatgtaatctcctaaatattccatcagctgctcagcagttatgatttccatcatcggtggaagtttcaccttccaggccaggagcaaaacattgaggatggccagcaaggggcagggtccgttctcattctgggtgatgatgggtgtgttctcttccttccactggatccacttgatgtgatacacagattgtcccgggaagcgttccttggaggccgccagcacctgagcggtctcctccccctcctcctccttgcacagaggaacagccccgggcaacaccgccgcgccctcctcctcctcagggaccctgttctccgctccctcctcactattgaactcgcagctactgggaaaagaatgcaggttagagaacgactccagagagtccaggctcggagattccccaggagggctcgggtcgctgcaactgctgctgaggccgccggcgctgctgggctcttcggagccggcggcggtcagttctgcttggcaggtgccggcgagatccgggcgggctcccgcgtctccggcggtacccaactcatgacccactccggccacggctgtctccggggaggcggtcaccttgtactgccctctcagaggcgcctcggcggcagcaggactctccaaaccactgtccttcaagtccaaacccgcggaggagctgcagggtccgggaacctcaggagagcccgcgggagaagccgagtccgggaggctcctcctggcggccgccgcccccagcccattcccgccgctggtctccgccgcccataccccaggaccatcaccagcggcgagcctggtctcctgtagcccttcctgcgaagaacctgtccctgacgctggcccggccgccaccccgtgttctagcggctgcaggctctcggggctgctctccataccgggccgcccgcccccagctctatggagaccgcggccacttctccgcagccagcgccttggacgccatgacagctgtattggcagcaacagcgccctggcgcggcctcggtcaggcacgtcaccggggagagtact

SEQ ID NO: 14082 - RNA, 7471 nt, Homo sapiens
  source 1..7471: mol_type = other RNA
gctgggattacaggcatgagccaccgcaccgggccagtttcctgactttttattttcagctataaaacaattatgagagccaaaggagccaggatcaccttccaaaacattttgttttgtccttctctaatttatgaggcattctttcttctcaaagcaggatattacagtgcagattaaaactggatattaaagttaatggtgacaaattattaagtagtttgaagaaatccttagaatatcagataaagagagacttaatggcagaagaagaagtctactggggttcaaagcttaggttttatatttctgccatggtatctcaacactttctctgggatagtacgatgccctaaaaaatacctgtgttaggcagacaagtctaaatctcctttctcaggacaataggacaaaactgaacttgaggcaatagttgaagaattttaccccgtttttcaagtttaattttcttgagatcagaaaagtaaaattagaaagtagaatccttcatgtaaaaaaatatatgcgtatcacaatttattaaactctaacatctaagagcaaaaacaccaggattaagtaagaacatgcatgaactaaaatttagatagatattcaaagtaagttaaatttaccagagtcctgcatctggcctctcccatgccattatcgctattttgcaatttgttttgttcaggaagcctctgattttaatatttaaagtgtcacctgagaagagtaacctcaattcttcatgttttctcaacaatcttagaggtgttggacatcattaataaaatatactaaattatcagagaacttaagaacgctaagattctgatgagttcctttaccattttcagtcactttctaaaagggatttaacttcacattatcaaataacattttacactaaaaacacaatttatatagccctaaaataatattacttgagagatctaaatgaattccaccaatgcaaacgaagtttatatactgtattagtaatttgataccaccgtattccatggagaaaaaggcaaagagaatctaaatatttagatctgtgaaagatactagaaaaaaatagatttttaaatgcttctgatcctctcaaaatactcttgattttgactctatagtctatagaacacacaaaaaactgtaaaatgcatttgggaagagatcacgccatactcaaagaaaattctacaaattttgacagcattaaaaaaactgacttaagatatattttgttattgagaaaaaagtgtgcacattcaagaacataggatgtgtaatatttgtgataaattaagtcatactttgtgcttatactatgccctttattcaggagtgcaaaacacttaatcaaaaagagcatccttcacatatttaaagagtacattgaggcacagaaagtttgcccaaggcaagatagaaagtcgggtttatagacacaaaatgatctagaattcttcatgtccaattccttaaaatacaaactgtagactatttgtaatgcctccatcttattttatcaaacattagtaattttactattataagtttatgcataagtactgtgtgataggtaatgcccataaggtttttatcatgttttaaggtaacttgtgcatggaataggaaaagttaatcaaatgtaatcaattcgcttttgctttttaacaaaacttaaataaatgagctatttgaggacagttctggaaattcttgccttgatttttctccaagattttagatatgtagttcacatgtgaacattaatatatgaacaattattttatttattggcctctagttctctttcctctcatgatctgtctcttagtgaattgactttctgattcattgaaagcaaaatgctaagaaggttttgtgcaagtgcaaaatgtttaatcttgggttcagtcaactagtctctgatactaacttgcttagttaagccaagatcaagaagtatgagaaagaacttgaaatatgataaagaatttgaaacagaatatgggataagtagtcaatatcagaaatgtgagacaataaaaacaagatatattccaaagcctaatcctaaatttaaatctacacttcattcaactctgaacctgaccttgaaacatggaagaagttactttacctaagcacactgcaccagtgtaaaaccaatgccaattttagctgctttatactgcttaatgtgtatatgtacacatgtattcttaaaatggtgattcttaaattgaagttctgaattcttttgagaatctaacagaggtcatgaaaacttgcttcagaaacacacatatgtaaagtacttttaagtgttgatcatgtactataaatcacagcattgtggatgcaatgggattagacatgaagaaaaattttatatttttaataaagactggttactaaccttaaggaatatacttagactctgaaagtaaaaggaaagtgcaatgaccatatttgttcattcatctgcctattttcaaatctaatgatgatttggttgatgcaaatatgtccctaatctaggctataaatgataaaaacaaaaatgtttaagttctaacttttgttagcagtatacatctaagaattttcaagtattacaaaatacttggaaggaaagactttaatataccactttcaaaatcctatgtacccaaaccagcaatgaagtggtgggatatataacgttaccttgggcaaaatttaagaaaataaagacacaatagctctaattttttttttttttttttttttgagacggagtctcgctctattgcccaggcttgcatgcagtggtgctatctcagctcactgcaatcactgcctcctgggttcaagcgattctcctgcctcagcctcccaagtagctgggatgacaggtgcccgccaccatgcctggctaattattgtatttttagtagagacagggttttgccatgttggccaggctggtctcgaactcctgatctcaggtgatccacctgcctcggcctcccaaagtactgggattacaggcatgatctaaattctttatacccttcaagggcaggaaaccagtatctctgaaaagcttgtttgttttaatacaattgaacatttcatctttccccccacagtaatcaaagcaaacattttatcattattattcttggtatatcaaagtaaattccaggaatgtaagaaagtctgacttggaaatattacatagaaaaaggctgaattaacacattacattttttagtttttccttgtaagtatacattgacatctacttatctgatagcagcactgctggttttgagtgagttttgttttgttttgtttccttccagagggaatgcagtatggcagcattttctttggaacaaattaagaagatagtaacaaataacagaagaaatacttctacacatatattttccatgggcaataaacagataagtatataattatgaaaaaatatgcctcaactatgctttttaaaatttctcaaggtatactggtttgtttttcttattcaaatataatgcactatcactactatctgtcccgggaaaaacaaaccctgaggtttgagttacctccttcagccaacagagtgatatcaagagtaaacttggattgaggtcaacctgtttgagccaatagagagttctgtagtatatctggttattttactaacgtatacatattctaggttataatcaagatactcattaaatattttctatcagagttttatatcccaaacaggttctttgatgatttatcatgctaccataggaaatttgaagaaataacaaattgtgtaacagaaatagacatgcaatataaaggacataaaagatacagcttgaccctggatttttcccttagaataattccttccataaataagactctatttttacatacagattcatcctataactggtcttggatcataaagttaatgacatagttgaaaaaatccagaccacacatttttgtggtcttttgtcaccccagaccacacacaaaaaaaacactctccaagtggatgctcaggtcagattatgatgctcttaaataaatgtactgaagcttagaatgtaaagcacacaactatttgcagcagcaatagtctttcaaaataactaaaacaaacttttaaatataaggcatataaaacagactattaaggatagttttccaaactatatatagaaacacaggaaaatatgtgtggcctcataataaagttaaataaatattatttctgagttcttataaacactatgaggttatagttttatttggttcccataaattaaaaactctgattgcttttacataaattcttagctactctcagacttttttttttttgagacggagtctccctctgtcacccaggctggagtgcagcagggcgatctcggctcactgcaacctctgcctgccgggttcaagcaattctcctgcctcagccctgagtagctgggactacaggcacgcaccaccatgccaggctgattttttgtatttttagtagagacagggtttcaccatgctggccaggctggtctcgaactcctggcctcagatgatccgcccaccttggcctcccaaaatgttgggattacaggcgtgagccactgcgcccggccctttcagatttttattaatgtctttttataagacacagagattatctctaacttcatttcagaaatgtgctttttcattggttttaataagtacatttaattttctagcaatgaacatgacttaaaatttaaggttcaaggtagttctagaaaaaggtagacactgaactatctgcttttctacatccccatatttacaaagcctagcatccactgtgctttcctccatacactcaatcacattgtcaataaatagtaactgtggtccaggttacctatgataaagactccaaaattcctcaaaattttacaacactacaaagtcattaatatctgatattgataggttataagtattagtgttatgtaactttttgctattggaaaagaaatacaaatctttatttttgctatctaaattaaaactaagctccatgatcaagataatacctaaaatgtacattcctaaataaaggtaaagctgtttaagggctgaactagtccaatatacaattaagggttatttattcctattcttttgtttttgtttttttgaatccctatgttaaacccgtggtttctcatgaattagatcataatttaacattgtaaaatttcagaaactattgtgctaatatttagatttcaggaaggaatcagactaaatcaattacctccattcattgttagaacagaagatataatagcttactaactgatatgagttatgaatgtcactatgacacaaaatttgctgtgatttgctaatctggctacaagtgcagtatttttcatgaatgtcaacacacagcatttccaacttgtaacatgaaactccagctcataaagagtgtattgtgtgacttgaaaaagtctgattgtaactaagtaacaaccgttcccctgaaaaaacgaacaaaatccattaggaaatcaggcacagacggtattgatcggtttttcttcctttcctcctgtggttttgtttctcaagacatataggtggttccaacagaagccaacacttgttacaaaataacacagctatttttttccttttctttttctttatctttttctcgtggttccttccgtttacgttcactattcccagattgtcttccacttgatggagaggcttgtgctggctggccctgctgagcctgtgtagaagcagcagcagcagcagctgctgcttgttcctgttcctgatagtattgagaagcccgtctgtcctcttcctcttggagtttctttgctagttccaaatcactgattccttccgggatttgttcccaattgatctcttggctctgctgttcttgttgtagagataatgccataagataatcctgatctatctgatcttgttgtcctttgtatacagtttcaggatctgaaggaggtcgaagatgaaattctgagtcacagaaatttccatcaccatctacgttgtgtaggctttcccaaacaactttctcttcagtaagaaacccctggtccgttaccaacaaatacagttgaccctgagggtctactaaccacccatggtacaaaggaatatcaagaagatcaaatactatgcattctggtgtatattcaaacactcgaacaccagtgaatcttacatttacatccaggcctgtctgtagtttgtgcaaaattgccatggcatcactcatattctgttcataatttaaacgttgaatttctgaaatttcttttggctttgcatcaagcatgtaatctcctaaatattccatcagctgctcagcagttatgatttccatcatcggtggaagtttcaccttccaggccaggagcaaaacattgaggatggccagcaaggggcagggtccgttctcattctgggtgatgatgggtgtgttctcttccttccactggatccacttgatgtgatacacagattgtcccgggaagcgttccttggaggccgccagcacctgagcggtctcctccccctcctcctccttgcacagaggaacagccccgggcaacaccgccgcgccctcctcctcctcagggaccctgttctccgctccctcctcactattgaactcgcagctactgggaaaagaatgcaggttagagaacgactccagagagtccaggctcggagattccccaggagggctcgggtcgctgcaactgctgctgaggccgccggcgctgctgggctcttcggagccggcggcggtcagttctgcttggcaggtgccggcgagatccgggcgggctcccgcgtctccggcggtacccaactcatgacccactccggccacggctgtctccggggaggcggtcaccttgtactgccctctcagaggcgcctcggcggcagcaggactctccaaaccactgtccttcaagtccaaacccgcggaggagctgcagggtccgggaacctcaggagagcccgcgggagaagccgagtccgggaggctcctcctggcggccgccgcccccagcccattcccgccgctggtctccgccgcccataccccaggaccatcaccagcggcgagcctggtctcctgtagcccttcctgcgaagaacctgtccctgacgctggcccggccgccaccccgtgttctagcggctgcaggctctcggggctgctctccataccgggccgcccgcccccagctctatggagaccgcggccacttctccgcagccagcgccttggacgccatgacagctgtattggcagcaacagcgccctggcgcggcctcggtcaggcacgtcaccggggagagtact

SEQ ID NO: 14083 - RNA, 7669 nt, Homo sapiens
  source 1..7669: mol_type = other RNA
gctgggattacaggcatgagccaccgcaccgggccagtttcctgactttttattttcagctataaaacaattatgagagccaaaggagccaggatcaccttccaaaacattttgttttgtccttctctaatttatgaggcattctttcttctcaaagcaggatattacagtgcagattaaaactggatattaaagttaatggtgacaaattattaagtagtttgaagaaatccttagaatatcagataaagagagacttaatggcagaagaagaagtctactggggttcaaagcttaggttttatatttctgccatggtatctcaacactttctctgggatagtacgatgccctaaaaaatacctgtgttaggcagacaagtctaaatctcctttctcaggacaataggacaaaactgaacttgaggcaatagttgaagaattttaccccgtttttcaagtttaattttcttgagatcagaaaagtaaaattagaaagtagaatccttcatgtaaaaaaatatatgcgtatcacaatttattaaactctaacatctaagagcaaaaacaccaggattaagtaagaacatgcatgaactaaaatttagatagatattcaaagtaagttaaatttaccagagtcctgcatctggcctctcccatgccattatcgctattttgcaatttgttttgttcaggaagcctctgattttaatatttaaagtgtcacctgagaagagtaacctcaattcttcatgttttctcaacaatcttagaggtgttggacatcattaataaaatatactaaattatcagagaacttaagaacgctaagattctgatgagttcctttaccattttcagtcactttctaaaagggatttaacttcacattatcaaataacattttacactaaaaacacaatttatatagccctaaaataatattacttgagagatctaaatgaattccaccaatgcaaacgaagtttatatactgtattagtaatttgataccaccgtattccatggagaaaaaggcaaagagaatctaaatatttagatctgtgaaagatactagaaaaaaatagatttttaaatgcttctgatcctctcaaaatactcttgattttgactctatagtctatagaacacacaaaaaactgtaaaatgcatttgggaagagatcacgccatactcaaagaaaattctacaaattttgacagcattaaaaaaactgacttaagatatattttgttattgagaaaaaagtgtgcacattcaagaacataggatgtgtaatatttgtgataaattaagtcatactttgtgcttatactatgccctttattcaggagtgcaaaacacttaatcaaaaagagcatccttcacatatttaaagagtacattgaggcacagaaagtttgcccaaggcaagatagaaagtcgggtttatagacacaaaatgatctagaattcttcatgtccaattccttaaaatacaaactgtagactatttgtaatgcctccatcttattttatcaaacattagtaattttactattataagtttatgcataagtactgtgtgataggtaatgcccataaggtttttatcatgttttaaggtaacttgtgcatggaataggaaaagttaatcaaatgtaatcaattcgcttttgctttttaacaaaacttaaataaatgagctatttgaggacagttctggaaattcttgccttgatttttctccaagattttagatatgtagttcacatgtgaacattaatatatgaacaattattttatttattggcctctagttctctttcctctcatgatctgtctcttagtgaattgactttctgattcattgaaagcaaaatgctaagaaggttttgtgcaagtgcaaaatgtttaatcttgggttcagtcaactagtctctgatactaacttgcttagttaagccaagatcaagaagtatgagaaagaacttgaaatatgataaagaatttgaaacagaatatgggataagtagtcaatatcagaaatgtgagacaataaaaacaagatatattccaaagcctaatcctaaatttaaatctacacttcattcaactctgaacctgaccttgaaacatggaagaagttactttacctaagcacactgcaccagtgtaaaaccaatgccaattttagctgctttatactgcttaatgtgtatatgtacacatgtattcttaaaatggtgattcttaaattgaagttctgaattcttttgagaatctaacagaggtcatgaaaacttgcttcagaaacacacatatgtaaagtacttttaagtgttgatcatgtactataaatcacagcattgtggatgcaatgggattagacatgaagaaaaattttatatttttaataaagactggttactaaccttaaggaatatacttagactctgaaagtaaaaggaaagtgcaatgaccatatttgttcattcatctgcctattttcaaatctaatgatgatttggttgatgcaaatatgtccctaatctaggctataaatgataaaaacaaaaatgtttaagttctaacttttgttagcagtatacatctaagaattttcaagtattacaaaatacttggaaggaaagactttaatataccactttcaaaatcctatgtacccaaaccagcaatgaagtggtgggatatataacgttaccttgggcaaaatttaagaaaataaagacacaatagctctaattttttttttttttttttttttgagacggagtctcgctctattgcccaggcttgcatgcagtggtgctatctcagctcactgcaatcactgcctcctgggttcaagcgattctcctgcctcagcctcccaagtagctgggatgacaggtgcccgccaccatgcctggctaattattgtatttttagtagagacagggttttgccatgttggccaggctggtctcgaactcctgatctcaggtgatccacctgcctcggcctcccaaagtactgggattacaggcatgatctaaattctttatacccttcaagggcaggaaaccagtatctctgaaaagcttgtttgttttaatacaattgaacatttcatctttccccccacagtaatcaaagcaaacattttatcattattattcttggtatatcaaagtaaattccaggaatgtaagaaagtctgacttggaaatattacatagaaaaaggctgaattaacacattacattttttagtttttccttgtaagtatacattgacatctacttatctgatagcagcactgctggttttgagtgagttttgttttgttttgtttccttccagagggaatgcagtatggcagcattttctttggaacaaattaagaagatagtaacaaataacagaagaaatacttctacacatatattttccatgggcaataaacagataagtatataattatgaaaaaatatgcctcaactatgctttttaaaatttctcaaggtatactggtttgtttttcttattcaaatataatgcactatcactactatctgtcccgggaaaaacaaaccctgaggtttgagttacctccttcagccaacagagtgatatcaagagtaaacttggattgaggtcaacctgtttgagccaatagagagttctgtagtatatctggttattttactaacgtatacatattctaggttataatcaagatactcattaaatattttctatcagagttttatatcccaaacaggttctttgatgatttatcatgctaccataggaaatttgaagaaataacaaattgtgtaacagaaatagacatgcaatataaaggacataaaagatacagcttgaccctggatttttcccttagaataattccttccataaataagactctatttttacatacagattcatcctataactggtcttggatcataaagttaatgacatagttgaaaaaatccagaccacacatttttgtggtcttttgtcaccccagaccacacacaaaaaaaacactctccaagtggatgctcaggtcagattatgatgctcttaaataaatgtactgaagcttagaatgtaaagcacacaactatttgcagcagcaatagtctttcaaaataactaaaacaaacttttaaatataaggcatataaaacagactattaaggatagttttccaaactatatatagaaacacaggaaaatatgtgtggcctcataataaagttaaataaatattatttctgagttcttataaacactatgaggttatagttttatttggttcccataaattaaaaactctgattgcttttacataaattcttagctactctcagacttttttttttttgagacggagtctccctctgtcacccaggctggagtgcagcagggcgatctcggctcactgcaacctctgcctgccgggttcaagcaattctcctgcctcagccctgagtagctgggactacaggcacgcaccaccatgccaggctgattttttgtatttttagtagagacagggtttcaccatgctggccaggctggtctcgaactcctggcctcagatgatccgcccaccttggcctcccaaaatgttgggattacaggcgtgagccactgcgcccggccctttcagatttttattaatgtctttttataagacacagagattatctctaacttcatttcagaaatgtgctttttcattggttttaataagtacatttaattttctagcaatgaacatgacttaaaatttaaggttcaaggtagttctagaaaaaggtagacactgaactatctgcttttctacatccccatatttacaaagcctagcatccactgtgctttcctccatacactcaatcacattgtcaataaatagtaactgtggtccaggttacctatgataaagactccaaaattcctcaaaattttacaacactacaaagtcattaatatctgatattgataggttataagtattagtgttatgtaactttttgctattggaaaagaaatacaaatctttatttttgctatctaaattaaaactaagctccatgatcaagataatacctaaaatgtacattcctaaataaaggtaaagctgtttaagggctgaactagtccaatatacaattaagggttatttattcctattcttttgtttttgtttttttgaatccctatgttaaacccgtggtttctcatgaattagatcataatttaacattgtaaaatttcagaaactattgtgctaatatttagatttcaggaaggaatcagactaaatcaattacctccattcattgttagaacagaagatataatagcttactaactgatatgagttatgaatgtcactatgacacaaaatttgctgtgatttgctaatctggctacaagtgcagtatttttcatgaatgtcaacacacagcatttccaacttgtaacatgaaactccagctcataaagagtgtattgtgtgacttgaaaaagtctgattgtaactaagtaacaaccgttcccctgaaaaaacgaacaaaatccattaggaaatcaggcacagacggtattgatcggtttttcttcctttcctcctgtggttttgtttctcaagacatataggtggttccaacagaagccaacacttgttacaaaataacacagctatttttttccttttctttttctttatctttttctcgtggttccttccgtttacgttcactattcccagattgtcttccacttgatggagaggcttgtgctggctggccctgctgagcctgtgtagaagcagcagcagcagcagctgctgcttgttcctgttcctgatagtattgagaagcccgtctgtcctcttcctcttggagtttctttgctagttccaaatcactgattccttccgggatttgttcccaattgatctcttggctctgctgttcttgttgtagagataatgccataagataatcctgatctatctgatcttgttgtcctttgtatacagtttcaggatctgaaggaggtcgaagatgaaattctgagtcacagaaatttccatcaccatctacgttgtgtaggctttcccaaacaactttctcttcagtaagaaacccctggtccgttaccaacaaatacagttgacccttgtatttggtcatggtgctaaaatgattattccgaaagaacacacaaagttctccttcctgaaccgttgaagttagttcacataatccatggtatgtcagttgagtggctgtgttatttagaaactgctcagctacaaagccttcactaaccagctcactattgtctgactgtttacaagagatgatcttctccactagttggttgtagctgcagttaccaacagcttttacaatgtcatcaatatttacatccaggcctgtctgtagtttgtgcaaaattgccatggcatcactcatattattttttcccttaagtgttttagaacttttcttaaatctacagcaatgatgaatctgttcataatttaaacgttgaatttctgaaatttcttttggctttgcatcaagcatgtaatctcctaaatattccatcagctgctcagcagttatgatttccatcatcggtggaagtttcaccttccaggccaggagcaaaacattgaggatggccagcaaggggcagggtccgttctcattctgggtgatgatgggtgtgttctcttccttccactggatccacttgatgtgatacacagattgtcccgggaagcgttccttggaggccgccagcacctgagcggtctcctccccctcctcctccttgcacagaggaacagccccgggcaacaccgccgcgccctcctcctcctcagggaccctgttctccgctccctcctcactattgaactcgcagctactgggaaaagaatgcaggttagagaacgactccagagagtccaggctcggagattccccaggagggctcgggtcgctgcaactgctgctgaggccgccggcgctgctgggctcttcggagccggcggcggtcagttctgcttggcaggtgccggcgagatccgggcgggctcccgcgtctccggcggtacccaactcatgacccactccggccacggctgtctccggggaggcggtcaccttgtactgccctctcagaggcgcctcggcggcagcaggactctccaaaccactgtccttcaagtccaaacccgcggaggagctgcagggtccgggaacctcaggagagcccgcgggagaagccgagtccgggaggctcctcctggcggccgccgcccccagcccattcccgccgctggtctccgccgcccataccccaggaccatcaccagcggcgagcctggtctcctgtagcccttcctgcgaagaacctgtccctgacgctggcccggccgccaccccgtgttctagcggctgcaggctctcggggctgctctccataccgggccgcccgcccccagctctatggagaccgcggccacttctccgcagccagcgccttggacgccatgacagctgtattggcagcaacagcgccctggcgcggcctcggtcaggcacgtcaccggggagagtact

SEQ ID NO: 14084 - RNA, 7615 nt, Homo sapiens
  source 1..7615: mol_type = other RNA
gctgggattacaggcatgagccaccgcaccgggccagtttcctgactttttattttcagctataaaacaattatgagagccaaaggagccaggatcaccttccaaaacattttgttttgtccttctctaatttatgaggcattctttcttctcaaagcaggatattacagtgcagattaaaactggatattaaagttaatggtgacaaattattaagtagtttgaagaaatccttagaatatcagataaagagagacttaatggcagaagaagaagtctactggggttcaaagcttaggttttatatttctgccatggtatctcaacactttctctgggatagtacgatgccctaaaaaatacctgtgttaggcagacaagtctaaatctcctttctcaggacaataggacaaaactgaacttgaggcaatagttgaagaattttaccccgtttttcaagtttaattttcttgagatcagaaaagtaaaattagaaagtagaatccttcatgtaaaaaaatatatgcgtatcacaatttattaaactctaacatctaagagcaaaaacaccaggattaagtaagaacatgcatgaactaaaatttagatagatattcaaagtaagttaaatttaccagagtcctgcatctggcctctcccatgccattatcgctattttgcaatttgttttgttcaggaagcctctgattttaatatttaaagtgtcacctgagaagagtaacctcaattcttcatgttttctcaacaatcttagaggtgttggacatcattaataaaatatactaaattatcagagaacttaagaacgctaagattctgatgagttcctttaccattttcagtcactttctaaaagggatttaacttcacattatcaaataacattttacactaaaaacacaatttatatagccctaaaataatattacttgagagatctaaatgaattccaccaatgcaaacgaagtttatatactgtattagtaatttgataccaccgtattccatggagaaaaaggcaaagagaatctaaatatttagatctgtgaaagatactagaaaaaaatagatttttaaatgcttctgatcctctcaaaatactcttgattttgactctatagtctatagaacacacaaaaaactgtaaaatgcatttgggaagagatcacgccatactcaaagaaaattctacaaattttgacagcattaaaaaaactgacttaagatatattttgttattgagaaaaaagtgtgcacattcaagaacataggatgtgtaatatttgtgataaattaagtcatactttgtgcttatactatgccctttattcaggagtgcaaaacacttaatcaaaaagagcatccttcacatatttaaagagtacattgaggcacagaaagtttgcccaaggcaagatagaaagtcgggtttatagacacaaaatgatctagaattcttcatgtccaattccttaaaatacaaactgtagactatttgtaatgcctccatcttattttatcaaacattagtaattttactattataagtttatgcataagtactgtgtgataggtaatgcccataaggtttttatcatgttttaaggtaacttgtgcatggaataggaaaagttaatcaaatgtaatcaattcgcttttgctttttaacaaaacttaaataaatgagctatttgaggacagttctggaaattcttgccttgatttttctccaagattttagatatgtagttcacatgtgaacattaatatatgaacaattattttatttattggcctctagttctctttcctctcatgatctgtctcttagtgaattgactttctgattcattgaaagcaaaatgctaagaaggttttgtgcaagtgcaaaatgtttaatcttgggttcagtcaactagtctctgatactaacttgcttagttaagccaagatcaagaagtatgagaaagaacttgaaatatgataaagaatttgaaacagaatatgggataagtagtcaatatcagaaatgtgagacaataaaaacaagatatattccaaagcctaatcctaaatttaaatctacacttcattcaactctgaacctgaccttgaaacatggaagaagttactttacctaagcacactgcaccagtgtaaaaccaatgccaattttagctgctttatactgcttaatgtgtatatgtacacatgtattcttaaaatggtgattcttaaattgaagttctgaattcttttgagaatctaacagaggtcatgaaaacttgcttcagaaacacacatatgtaaagtacttttaagtgttgatcatgtactataaatcacagcattgtggatgcaatgggattagacatgaagaaaaattttatatttttaataaagactggttactaaccttaaggaatatacttagactctgaaagtaaaaggaaagtgcaatgaccatatttgttcattcatctgcctattttcaaatctaatgatgatttggttgatgcaaatatgtccctaatctaggctataaatgataaaaacaaaaatgtttaagttctaacttttgttagcagtatacatctaagaattttcaagtattacaaaatacttggaaggaaagactttaatataccactttcaaaatcctatgtacccaaaccagcaatgaagtggtgggatatataacgttaccttgggcaaaatttaagaaaataaagacacaatagctctaattttttttttttttttttttttgagacggagtctcgctctattgcccaggcttgcatgcagtggtgctatctcagctcactgcaatcactgcctcctgggttcaagcgattctcctgcctcagcctcccaagtagctgggatgacaggtgcccgccaccatgcctggctaattattgtatttttagtagagacagggttttgccatgttggccaggctggtctcgaactcctgatctcaggtgatccacctgcctcggcctcccaaagtactgggattacaggcatgatctaaattctttatacccttcaagggcaggaaaccagtatctctgaaaagcttgtttgttttaatacaattgaacatttcatctttccccccacagtaatcaaagcaaacattttatcattattattcttggtatatcaaagtaaattccaggaatgtaagaaagtctgacttggaaatattacatagaaaaaggctgaattaacacattacattttttagtttttccttgtaagtatacattgacatctacttatctgatagcagcactgctggttttgagtgagttttgttttgttttgtttccttccagagggaatgcagtatggcagcattttctttggaacaaattaagaagatagtaacaaataacagaagaaatacttctacacatatattttccatgggcaataaacagataagtatataattatgaaaaaatatgcctcaactatgctttttaaaatttctcaaggtatactggtttgtttttcttattcaaatataatgcactatcactactatctgtcccgggaaaaacaaaccctgaggtttgagttacctccttcagccaacagagtgatatcaagagtaaacttggattgaggtcaacctgtttgagccaatagagagttctgtagtatatctggttattttactaacgtatacatattctaggttataatcaagatactcattaaatattttctatcagagttttatatcccaaacaggttctttgatgatttatcatgctaccataggaaatttgaagaaataacaaattgtgtaacagaaatagacatgcaatataaaggacataaaagatacagcttgaccctggatttttcccttagaataattccttccataaataagactctatttttacatacagattcatcctataactggtcttggatcataaagttaatgacatagttgaaaaaatccagaccacacatttttgtggtcttttgtcaccccagaccacacacaaaaaaaacactctccaagtggatgctcaggtcagattatgatgctcttaaataaatgtactgaagcttagaatgtaaagcacacaactatttgcagcagcaatagtctttcaaaataactaaaacaaacttttaaatataaggcatataaaacagactattaaggatagttttccaaactatatatagaaacacaggaaaatatgtgtggcctcataataaagttaaataaatattatttctgagttcttataaacactatgaggttatagttttatttggttcccataaattaaaaactctgattgcttttacataaattcttagctactctcagacttttttttttttgagacggagtctccctctgtcacccaggctggagtgcagcagggcgatctcggctcactgcaacctctgcctgccgggttcaagcaattctcctgcctcagccctgagtagctgggactacaggcacgcaccaccatgccaggctgattttttgtatttttagtagagacagggtttcaccatgctggccaggctggtctcgaactcctggcctcagatgatccgcccaccttggcctcccaaaatgttgggattacaggcgtgagccactgcgcccggccctttcagatttttattaatgtctttttataagacacagagattatctctaacttcatttcagaaatgtgctttttcattggttttaataagtacatttaattttctagcaatgaacatgacttaaaatttaaggttcaaggtagttctagaaaaaggtagacactgaactatctgcttttctacatccccatatttacaaagcctagcatccactgtgctttcctccatacactcaatcacattgtcaataaatagtaactgtggtccaggttacctatgataaagactccaaaattcctcaaaattttacaacactacaaagtcattaatatctgatattgataggttataagtattagtgttatgtaactttttgctattggaaaagaaatacaaatctttatttttgctatctaaattaaaactaagctccatgatcaagataatacctaaaatgtacattcctaaataaaggtaaagctgtttaagggctgaactagtccaatatacaattaagggttatttattcctattcttttgtttttgtttttttgaatccctatgttaaacccgtggtttctcatgaattagatcataatttaacattgtaaaatttcagaaactattgtgctaatatttagatttcaggaaggaatcagactaaatcaattacctccattcattgttagaacagaagatataatagcttactaactgatatgagttatgaatgtcactatgacacaaaatttgctgtgatttgctaatctggctacaagtgcagtatttttcatgaatgtcaacacacagcatttccaacttgtaacatgaaactccagctcataaagagtgtattgtgtgacttgaaaaagtctgattgtaactaagtaacaaccgttcccctgaaaaaacgaacaaaatccattaggaaatcaggcacagacggtattgatcggtttttcttcctttcctcctgtggttttgtttctcaagacatataggtggttccaacagaagccaacacttgttacaaaataacacagctatttttttccttttctttttctttatctttttctcgtggttccttccgtttacgttcactattcccagattgtcttccacttgatggagaggcttgtgctggctggccctgctgagcctgtgtagaagcagcagcagcagcagctgctgcttgttcctgttcctgatagtattgagaagcccgtctgtcctcttcctcttggagtttctttgctagttccaaatcactgattccttccgggatttgttcccaattgatctcttggctctgctgttcttgttgtagagataatgccataagataatcctgatctatctgatcttgttgtcctttgtatacagtttcaggatctgaaggaggtcgaagatgaaattctgagtcacagaaatttccatcaccatctacgttgtgtaggctttcccaaacaactttctcttcagtaagaaacccctggtccgttaccaacaaatacagttgacccttgtatttggtcatggtgctaaaatgattattccgaaagaacacacaaagttctccttcctgaaccgttgaagttagttcacataatccatggtatgtcagttgagtggctgtgttatttagaaactgctcagctacaaagccttcactaaccagctcactattgtctgactgtttacaagagatgatcttctccactagttggttgtagctgcagttaccaacagcttttacaatgtcatcaatatttacatccaggcctgtctgtagtttgtgcaaaattgccatggcatcactcatattctgttcataatttaaacgttgaatttctgaaatttcttttggctttgcatcaagcatgtaatctcctaaatattccatcagctgctcagcagttatgatttccatcatcggtggaagtttcaccttccaggccaggagcaaaacattgaggatggccagcaaggggcagggtccgttctcattctgggtgatgatgggtgtgttctcttccttccactggatccacttgatgtgatacacagattgtcccgggaagcgttccttggaggccgccagcacctgagcggtctcctccccctcctcctccttgcacagaggaacagccccgggcaacaccgccgcgccctcctcctcctcagggaccctgttctccgctccctcctcactattgaactcgcagctactgggaaaagaatgcaggttagagaacgactccagagagtccaggctcggagattccccaggagggctcgggtcgctgcaactgctgctgaggccgccggcgctgctgggctcttcggagccggcggcggtcagttctgcttggcaggtgccggcgagatccgggcgggctcccgcgtctccggcggtacccaactcatgacccactccggccacggctgtctccggggaggcggtcaccttgtactgccctctcagaggcgcctcggcggcagcaggactctccaaaccactgtccttcaagtccaaacccgcggaggagctgcagggtccgggaacctcaggagagcccgcgggagaagccgagtccgggaggctcctcctggcggccgccgcccccagcccattcccgccgctggtctccgccgcccataccccaggaccatcaccagcggcgagcctggtctcctgtagcccttcctgcgaagaacctgtccctgacgctggcccggccgccaccccgtgttctagcggctgcaggctctcggggctgctctccataccgggccgcccgcccccagctctatggagaccgcggccacttctccgcagccagcgccttggacgccatgacagctgtattggcagcaacagcgccctggcgcggcctcggtcaggcacgtcaccggggagagtact

SEQ ID NO: 14085 - RNA, 7771 nt, Homo sapiens
  source 1..7771: mol_type = other RNA
gctgggattacaggcatgagccaccgcaccgggccagtttcctgactttttattttcagctataaaacaattatgagagccaaaggagccaggatcaccttccaaaacattttgttttgtccttctctaatttatgaggcattctttcttctcaaagcaggatattacagtgcagattaaaactggatattaaagttaatggtgacaaattattaagtagtttgaagaaatccttagaatatcagataaagagagacttaatggcagaagaagaagtctactggggttcaaagcttaggttttatatttctgccatggtatctcaacactttctctgggatagtacgatgccctaaaaaatacctgtgttaggcagacaagtctaaatctcctttctcaggacaataggacaaaactgaacttgaggcaatagttgaagaattttaccccgtttttcaagtttaattttcttgagatcagaaaagtaaaattagaaagtagaatccttcatgtaaaaaaatatatgcgtatcacaatttattaaactctaacatctaagagcaaaaacaccaggattaagtaagaacatgcatgaactaaaatttagatagatattcaaagtaagttaaatttaccagagtcctgcatctggcctctcccatgccattatcgctattttgcaatttgttttgttcaggaagcctctgattttaatatttaaagtgtcacctgagaagagtaacctcaattcttcatgttttctcaacaatcttagaggtgttggacatcattaataaaatatactaaattatcagagaacttaagaacgctaagattctgatgagttcctttaccattttcagtcactttctaaaagggatttaacttcacattatcaaataacattttacactaaaaacacaatttatatagccctaaaataatattacttgagagatctaaatgaattccaccaatgcaaacgaagtttatatactgtattagtaatttgataccaccgtattccatggagaaaaaggcaaagagaatctaaatatttagatctgtgaaagatactagaaaaaaatagatttttaaatgcttctgatcctctcaaaatactcttgattttgactctatagtctatagaacacacaaaaaactgtaaaatgcatttgggaagagatcacgccatactcaaagaaaattctacaaattttgacagcattaaaaaaactgacttaagatatattttgttattgagaaaaaagtgtgcacattcaagaacataggatgtgtaatatttgtgataaattaagtcatactttgtgcttatactatgccctttattcaggagtgcaaaacacttaatcaaaaagagcatccttcacatatttaaagagtacattgaggcacagaaagtttgcccaaggcaagatagaaagtcgggtttatagacacaaaatgatctagaattcttcatgtccaattccttaaaatacaaactgtagactatttgtaatgcctccatcttattttatcaaacattagtaattttactattataagtttatgcataagtactgtgtgataggtaatgcccataaggtttttatcatgttttaaggtaacttgtgcatggaataggaaaagttaatcaaatgtaatcaattcgcttttgctttttaacaaaacttaaataaatgagctatttgaggacagttctggaaattcttgccttgatttttctccaagattttagatatgtagttcacatgtgaacattaatatatgaacaattattttatttattggcctctagttctctttcctctcatgatctgtctcttagtgaattgactttctgattcattgaaagcaaaatgctaagaaggttttgtgcaagtgcaaaatgtttaatcttgggttcagtcaactagtctctgatactaacttgcttagttaagccaagatcaagaagtatgagaaagaacttgaaatatgataaagaatttgaaacagaatatgggataagtagtcaatatcagaaatgtgagacaataaaaacaagatatattccaaagcctaatcctaaatttaaatctacacttcattcaactctgaacctgaccttgaaacatggaagaagttactttacctaagcacactgcaccagtgtaaaaccaatgccaattttagctgctttatactgcttaatgtgtatatgtacacatgtattcttaaaatggtgattcttaaattgaagttctgaattcttttgagaatctaacagaggtcatgaaaacttgcttcagaaacacacatatgtaaagtacttttaagtgttgatcatgtactataaatcacagcattgtggatgcaatgggattagacatgaagaaaaattttatatttttaataaagactggttactaaccttaaggaatatacttagactctgaaagtaaaaggaaagtgcaatgaccatatttgttcattcatctgcctattttcaaatctaatgatgatttggttgatgcaaatatgtccctaatctaggctataaatgataaaaacaaaaatgtttaagttctaacttttgttagcagtatacatctaagaattttcaagtattacaaaatacttggaaggaaagactttaatataccactttcaaaatcctatgtacccaaaccagcaatgaagtggtgggatatataacgttaccttgggcaaaatttaagaaaataaagacacaatagctctaattttttttttttttttttttttgagacggagtctcgctctattgcccaggcttgcatgcagtggtgctatctcagctcactgcaatcactgcctcctgggttcaagcgattctcctgcctcagcctcccaagtagctgggatgacaggtgcccgccaccatgcctggctaattattgtatttttagtagagacagggttttgccatgttggccaggctggtctcgaactcctgatctcaggtgatccacctgcctcggcctcccaaagtactgggattacaggcatgatctaaattctttatacccttcaagggcaggaaaccagtatctctgaaaagcttgtttgttttaatacaattgaacatttcatctttccccccacagtaatcaaagcaaacattttatcattattattcttggtatatcaaagtaaattccaggaatgtaagaaagtctgacttggaaatattacatagaaaaaggctgaattaacacattacattttttagtttttccttgtaagtatacattgacatctacttatctgatagcagcactgctggttttgagtgagttttgttttgttttgtttccttccagagggaatgcagtatggcagcattttctttggaacaaattaagaagatagtaacaaataacagaagaaatacttctacacatatattttccatgggcaataaacagataagtatataattatgaaaaaatatgcctcaactatgctttttaaaatttctcaaggtatactggtttgtttttcttattcaaatataatgcactatcactactatctgtcccgggaaaaacaaaccctgaggtttgagttacctccttcagccaacagagtgatatcaagagtaaacttggattgaggtcaacctgtttgagccaatagagagttctgtagtatatctggttattttactaacgtatacatattctaggttataatcaagatactcattaaatattttctatcagagttttatatcccaaacaggttctttgatgatttatcatgctaccataggaaatttgaagaaataacaaattgtgtaacagaaatagacatgcaatataaaggacataaaagatacagcttgaccctggatttttcccttagaataattccttccataaataagactctatttttacatacagattcatcctataactggtcttggatcataaagttaatgacatagttgaaaaaatccagaccacacatttttgtggtcttttgtcaccccagaccacacacaaaaaaaacactctccaagtggatgctcaggtcagattatgatgctcttaaataaatgtactgaagcttagaatgtaaagcacacaactatttgcagcagcaatagtctttcaaaataactaaaacaaacttttaaatataaggcatataaaacagactattaaggatagttttccaaactatatatagaaacacaggaaaatatgtgtggcctcataataaagttaaataaatattatttctgagttcttataaacactatgaggttatagttttatttggttcccataaattaaaaactctgattgcttttacataaattcttagctactctcagacttttttttttttgagacggagtctccctctgtcacccaggctggagtgcagcagggcgatctcggctcactgcaacctctgcctgccgggttcaagcaattctcctgcctcagccctgagtagctgggactacaggcacgcaccaccatgccaggctgattttttgtatttttagtagagacagggtttcaccatgctggccaggctggtctcgaactcctggcctcagatgatccgcccaccttggcctcccaaaatgttgggattacaggcgtgagccactgcgcccggccctttcagatttttattaatgtctttttataagacacagagattatctctaacttcatttcagaaatgtgctttttcattggttttaataagtacatttaattttctagcaatgaacatgacttaaaatttaaggttcaaggtagttctagaaaaaggtagacactgaactatctgcttttctacatccccatatttacaaagcctagcatccactgtgctttcctccatacactcaatcacattgtcaataaatagtaactgtggtccaggttacctatgataaagactccaaaattcctcaaaattttacaacactacaaagtcattaatatctgatattgataggttataagtattagtgttatgtaactttttgctattggaaaagaaatacaaatctttatttttgctatctaaattaaaactaagctccatgatcaagataatacctaaaatgtacattcctaaataaaggtaaagctgtttaagggctgaactagtccaatatacaattaagggttatttattcctattcttttgtttttgtttttttgaatccctatgttaaacccgtggtttctcatgaattagatcataatttaacattgtaaaatttcagaaactattgtgctaatatttagatttcaggaaggaatcagactaaatcaattacctccattcattgttagaacagaagatataatagcttactaactgatatgagttatgaatgtcactatgacacaaaatttgctgtgatttgctaatctggctacaagtgcagtatttttcatgaatgtcaacacacagcatttccaacttgtaacatgaaactccagctcataaagagtgtattgtgtgacttgaaaaagtctgattgtaactaagtaacaaccgttcccctgaaaaaacgaacaaaatccattaggaaatcaggcacagacggtattgatcggtttttcttcctttcctcctgtggttttgtttctcaagacatataggtggttccaacagaagccaacacttgttacaaaataacacagctatttttttccttttctttttctttatctttttctcgtggttccttccgtttacgttcactattcccagattgtcttccacttgatggagaggcttgtgctggctggccctgctgagcctgtgtagaagcagcagcagcagcagctgctgcttgttcctgttcctgatagtattgagaagcccgtctgtcctcttcctcttggagtttctttgctagttccaaatcactgattccttccgggatttgttcccaattgatctcttggctctgctgttcttgttgtagagataatgccataagataatcctgatctatctgatcttgttgtcctttgtatacagtttcaggatctgaaggaggtcgaagatgaaattctgagtcacagaaatttccatcaccatctacgttgtgtaggctttcccaaacaactttctcttcagtaagaaacccctggtccgttaccaacaaatacagttgacccttgtatttggtcatggtgctaaaatgattattccgaaagaacacacaaagttctccttcctgaaccgttgaagttagttcacataatccatggtatgtcagttgagtggctgtgttatttagaaactgctcagctacaaagccttcactaaccagctcactattgtctgactgtttacaagagatgatcttctccactagttggttgtagctgcagttaccaacagcttttacaatgtcatcaatctgagggtctactaaccacccatggtacaaaggaatatcaagaagatcaaatactatgcattctggtgtatattcaaacactcgaacaccagtgaatcttacatttacatccaggcctgtctgtagtttgtgcaaaattgccatggcatcactcatattattttttcccttaagtgttttagaacttttcttaaatctacagcaatgatgaatctgttcataatttaaacgttgaatttctgaaatttcttttggctttgcatcaagcatgtaatctcctaaatattccatcagctgctcagcagttatgatttccatcatcggtggaagtttcaccttccaggccaggagcaaaacattgaggatggccagcaaggggcagggtccgttctcattctgggtgatgatgggtgtgttctcttccttccactggatccacttgatgtgatacacagattgtcccgggaagcgttccttggaggccgccagcacctgagcggtctcctccccctcctcctccttgcacagaggaacagccccgggcaacaccgccgcgccctcctcctcctcagggaccctgttctccgctccctcctcactattgaactcgcagctactgggaaaagaatgcaggttagagaacgactccagagagtccaggctcggagattccccaggagggctcgggtcgctgcaactgctgctgaggccgccggcgctgctgggctcttcggagccggcggcggtcagttctgcttggcaggtgccggcgagatccgggcgggctcccgcgtctccggcggtacccaactcatgacccactccggccacggctgtctccggggaggcggtcaccttgtactgccctctcagaggcgcctcggcggcagcaggactctccaaaccactgtccttcaagtccaaacccgcggaggagctgcagggtccgggaacctcaggagagcccgcgggagaagccgagtccgggaggctcctcctggcggccgccgcccccagcccattcccgccgctggtctccgccgcccataccccaggaccatcaccagcggcgagcctggtctcctgtagcccttcctgcgaagaacctgtccctgacgctggcccggccgccaccccgtgttctagcggctgcaggctctcggggctgctctccataccgggccgcccgcccccagctctatggagaccgcggccacttctccgcagccagcgccttggacgccatgacagctgtattggcagcaacagcgccctggcgcggcctcggtcaggcacgtcaccggggagagtact

SEQ ID NO: 14086 - RNA, 7673 nt, Homo sapiens
  source 1..7673: mol_type = other RNA
gctgggattacaggcatgagccaccgcaccgggccagtttcctgactttttattttcagctataaaacaattatgagagccaaaggagccaggatcaccttccaaaacattttgttttgtccttctctaatttatgaggcattctttcttctcaaagcaggatattacagtgcagattaaaactggatattaaagttaatggtgacaaattattaagtagtttgaagaaatccttagaatatcagataaagagagacttaatggcagaagaagaagtctactggggttcaaagcttaggttttatatttctgccatggtatctcaacactttctctgggatagtacgatgccctaaaaaatacctgtgttaggcagacaagtctaaatctcctttctcaggacaataggacaaaactgaacttgaggcaatagttgaagaattttaccccgtttttcaagtttaattttcttgagatcagaaaagtaaaattagaaagtagaatccttcatgtaaaaaaatatatgcgtatcacaatttattaaactctaacatctaagagcaaaaacaccaggattaagtaagaacatgcatgaactaaaatttagatagatattcaaagtaagttaaatttaccagagtcctgcatctggcctctcccatgccattatcgctattttgcaatttgttttgttcaggaagcctctgattttaatatttaaagtgtcacctgagaagagtaacctcaattcttcatgttttctcaacaatcttagaggtgttggacatcattaataaaatatactaaattatcagagaacttaagaacgctaagattctgatgagttcctttaccattttcagtcactttctaaaagggatttaacttcacattatcaaataacattttacactaaaaacacaatttatatagccctaaaataatattacttgagagatctaaatgaattccaccaatgcaaacgaagtttatatactgtattagtaatttgataccaccgtattccatggagaaaaaggcaaagagaatctaaatatttagatctgtgaaagatactagaaaaaaatagatttttaaatgcttctgatcctctcaaaatactcttgattttgactctatagtctatagaacacacaaaaaactgtaaaatgcatttgggaagagatcacgccatactcaaagaaaattctacaaattttgacagcattaaaaaaactgacttaagatatattttgttattgagaaaaaagtgtgcacattcaagaacataggatgtgtaatatttgtgataaattaagtcatactttgtgcttatactatgccctttattcaggagtgcaaaacacttaatcaaaaagagcatccttcacatatttaaagagtacattgaggcacagaaagtttgcccaaggcaagatagaaagtcgggtttatagacacaaaatgatctagaattcttcatgtccaattccttaaaatacaaactgtagactatttgtaatgcctccatcttattttatcaaacattagtaattttactattataagtttatgcataagtactgtgtgataggtaatgcccataaggtttttatcatgttttaaggtaacttgtgcatggaataggaaaagttaatcaaatgtaatcaattcgcttttgctttttaacaaaacttaaataaatgagctatttgaggacagttctggaaattcttgccttgatttttctccaagattttagatatgtagttcacatgtgaacattaatatatgaacaattattttatttattggcctctagttctctttcctctcatgatctgtctcttagtgaattgactttctgattcattgaaagcaaaatgctaagaaggttttgtgcaagtgcaaaatgtttaatcttgggttcagtcaactagtctctgatactaacttgcttagttaagccaagatcaagaagtatgagaaagaacttgaaatatgataaagaatttgaaacagaatatgggataagtagtcaatatcagaaatgtgagacaataaaaacaagatatattccaaagcctaatcctaaatttaaatctacacttcattcaactctgaacctgaccttgaaacatggaagaagttactttacctaagcacactgcaccagtgtaaaaccaatgccaattttagctgctttatactgcttaatgtgtatatgtacacatgtattcttaaaatggtgattcttaaattgaagttctgaattcttttgagaatctaacagaggtcatgaaaacttgcttcagaaacacacatatgtaaagtacttttaagtgttgatcatgtactataaatcacagcattgtggatgcaatgggattagacatgaagaaaaattttatatttttaataaagactggttactaaccttaaggaatatacttagactctgaaagtaaaaggaaagtgcaatgaccatatttgttcattcatctgcctattttcaaatctaatgatgatttggttgatgcaaatatgtccctaatctaggctataaatgataaaaacaaaaatgtttaagttctaacttttgttagcagtatacatctaagaattttcaagtattacaaaatacttggaaggaaagactttaatataccactttcaaaatcctatgtacccaaaccagcaatgaagtggtgggatatataacgttaccttgggcaaaatttaagaaaataaagacacaatagctctaattttttttttttttttttttttgagacggagtctcgctctattgcccaggcttgcatgcagtggtgctatctcagctcactgcaatcactgcctcctgggttcaagcgattctcctgcctcagcctcccaagtagctgggatgacaggtgcccgccaccatgcctggctaattattgtatttttagtagagacagggttttgccatgttggccaggctggtctcgaactcctgatctcaggtgatccacctgcctcggcctcccaaagtactgggattacaggcatgatctaaattctttatacccttcaagggcaggaaaccagtatctctgaaaagcttgtttgttttaatacaattgaacatttcatctttccccccacagtaatcaaagcaaacattttatcattattattcttggtatatcaaagtaaattccaggaatgtaagaaagtctgacttggaaatattacatagaaaaaggctgaattaacacattacattttttagtttttccttgtaagtatacattgacatctacttatctgatagcagcactgctggttttgagtgagttttgttttgttttgtttccttccagagggaatgcagtatggcagcattttctttggaacaaattaagaagatagtaacaaataacagaagaaatacttctacacatatattttccatgggcaataaacagataagtatataattatgaaaaaatatgcctcaactatgctttttaaaatttctcaaggtatactggtttgtttttcttattcaaatataatgcactatcactactatctgtcccgggaaaaacaaaccctgaggtttgagttacctccttcagccaacagagtgatatcaagagtaaacttggattgaggtcaacctgtttgagccaatagagagttctgtagtatatctggttattttactaacgtatacatattctaggttataatcaagatactcattaaatattttctatcagagttttatatcccaaacaggttctttgatgatttatcatgctaccataggaaatttgaagaaataacaaattgtgtaacagaaatagacatgcaatataaaggacataaaagatacagcttgaccctggatttttcccttagaataattccttccataaataagactctatttttacatacagattcatcctataactggtcttggatcataaagttaatgacatagttgaaaaaatccagaccacacatttttgtggtcttttgtcaccccagaccacacacaaaaaaaacactctccaagtggatgctcaggtcagattatgatgctcttaaataaatgtactgaagcttagaatgtaaagcacacaactatttgcagcagcaatagtctttcaaaataactaaaacaaacttttaaatataaggcatataaaacagactattaaggatagttttccaaactatatatagaaacacaggaaaatatgtgtggcctcataataaagttaaataaatattatttctgagttcttataaacactatgaggttatagttttatttggttcccataaattaaaaactctgattgcttttacataaattcttagctactctcagacttttttttttttgagacggagtctccctctgtcacccaggctggagtgcagcagggcgatctcggctcactgcaacctctgcctgccgggttcaagcaattctcctgcctcagccctgagtagctgggactacaggcacgcaccaccatgccaggctgattttttgtatttttagtagagacagggtttcaccatgctggccaggctggtctcgaactcctggcctcagatgatccgcccaccttggcctcccaaaatgttgggattacaggcgtgagccactgcgcccggccctttcagatttttattaatgtctttttataagacacagagattatctctaacttcatttcagaaatgtgctttttcattggttttaataagtacatttaattttctagcaatgaacatgacttaaaatttaaggttcaaggtagttctagaaaaaggtagacactgaactatctgcttttctacatccccatatttacaaagcctagcatccactgtgctttcctccatacactcaatcacattgtcaataaatagtaactgtggtccaggttacctatgataaagactccaaaattcctcaaaattttacaacactacaaagtcattaatatctgatattgataggttataagtattagtgttatgtaactttttgctattggaaaagaaatacaaatctttatttttgctatctaaattaaaactaagctccatgatcaagataatacctaaaatgtacattcctaaataaaggtaaagctgtttaagggctgaactagtccaatatacaattaagggttatttattcctattcttttgtttttgtttttttgaatccctatgttaaacccgtggtttctcatgaattagatcataatttaacattgtaaaatttcagaaactattgtgctaatatttagatttcaggaaggaatcagactaaatcaattacctccattcattgttagaacagaagatataatagcttactaactgatatgagttatgaatgtcactatgacacaaaatttgctgtgatttgctaatctggctacaagtgcagtatttttcatgaatgtcaacacacagcatttccaacttgtaacatgaaactccagctcataaagagtgtattgtgtgacttgaaaaagtctgattgtaactaagtaacaaccgttcccctgaaaaaacgaacaaaatccattaggaaatcaggcacagacggtattgatcggtttttcttcctttcctcctgtggttttgtttctcaagacatataggtggttccaacagaagccaacacttgttacaaaataacacagctatttttttccttttctttttctttatctttttctcgtggttccttccgtttacgttcactattcccagattgtcttccacttgatggagaggcttgtgctggctggccctgctgagcctgtgtagaagcagcagcagcagcagctgctgcttgttcctgttcctgatagtattgagaagcccgtctgtcctcttcctcttggagtttctttgctagttccaaatcactgattccttccgggatttgttcccaattgatctcttggctctgctgttcttgttgtagagataatgccataagataatcctgatctatctgatcttgttgtcctttgtatacagtttcaggatctgaaggaggtcgaagatgaaattctgagtcacagaaatttccatcaccatctacgttgtgtaggctttcccaaacaactttctcttcagtaagaaacccctggtccgttaccaacaaatacagttgacccttgtatttggtcatggtgctaaaatgattattccgaaagaacacacaaagttctccttcctgaaccgttgaagttagttcacataatccatggtatgtcagttgagtggctgtgttatttagaaactgctcagctacaaagccttcactaaccagctcactattgtctgactgtttacaagagatgatcttctccactagttggttgtagctgcagttaccaacagcttttacaatgtcatcaatctgagggtctactaaccacccatggtacaaaggaatatcaagaagatcaaatactatgcattctggtgtatattcaaacactcgaacaccagtgaatcttacatttacatccaggcctgtctgtagtttgtgcaaaattgccatggcatcactcatattctgttcataatttaaacgttgaatttctgaaatttcttttggctttgcatcaagcatgtaatctcctaaatattccatcagctgctcagcagttatgatttccatcatcggtggaagtttcaccttccaggccaggagcaaaacattgaggatggccagcaaggggcagggtccgttctcattctgggtgatgatgggtgtgttctcttccttccactggatccacttgatgtgatacacagattgtcccgggaagcgttccttggaggccgccagcacctgagcggtctcctccccctcctcctccttgcacagaggaacagccccgggcaacaccgccgcgccctcctcctcctcagggaccctgttctccgctccctcctcactattgaactcgcagctactgggaaaagaatgcaggttagagaacgactccagagagtccaggctcggagattccccaggagggctcgggtcgctgcaactgctgctgaggccgccggcgctgctgggctcttcggagccggcggcggtcagttctgcttggcaggtgccggcgagatccgggcgggctcccgcgtctccggcggtacccaactcatgacccactccggccacggctgtctccggggaggcggtcaccttgtactgccctctcagaggcgcctcggcggcagcaggactctccaaaccactgtccttcaagtccaaacccgcggaggagctgcagggtccgggaacctcaggagagcccgcgggagaagccgagtccgggaggctcctcctggcggccgccgcccccagcccattcccgccgctggtctccgccgcccataccccaggaccatcaccagcggcgagcctggtctcctgtagcccttcctgcgaagaacctgtccctgacgctggcccggccgccaccccgtgttctagcggctgcaggctctcggggctgctctccataccgggccgcccgcccccagctctatggagaccgcggccacttctccgcagccagcgccttggacgccatgacagctgtattggcagcaacagc

SEQ ID NO: 14087 - RNA, 6767 nt, Homo sapiens
  source 1..6767: mol_type = other RNA
gctgggattacaggcatgagccaccgcaccgggcctgccaaggcaattttagattgagcaagtgcagagccctttgcgcaggacccctggcatctgcccagcatgcctggctgtattctcttttttttggagacatagtctcactttgtcacccaggctggctggagtgcagtggcatgatcttggctcactgcaacctccacctcctgggttcaagcaactcctgtgcctcagcctcctgagtagttgggattataggcacgcaccaccatgcccagctaatatttgtatttttagtagaaacaaacagggtttcaccatgttggccaagctggtctccaacccctgacctcaggtgatccgcccaccttggcctcccaaagtgctgggattacaggcatgagccactgtgcccagccctggctgtattcttgaagctgcccggggaaggctcacgaagggaggagcatctggttgtacctgattctggagacagcattttacctgcccctttacccactgtactccatccaaaatgaccctgcagtgccctgcagaggtctcaggccttggcctagagaacagagggctttgctcgtgctccccgctctgtctgcagtgctcttcctcttctatagccactcgaccatatctaggaatgcccagctcagtctacctctgaccctcacagtcctgttgacctgaggttctggatcagtgtccccacaaagcccagtcgtgttgccaagtgatgggtgtaggcgccagcactgtggcacttgctgagagtggcatatgattttttgcaggtcctagccctgggggtagcccagacacccccccagtgctgacaggttatgtgctgtggagggtgctgaaatggtttctcctccagtgggctggaatcacagatgggctgtttacggagcaagtgccggctccaccccatgagatctgggggttagagatgagcaggatgagtcctttgtaactgagaatgaagctgtacccctttctctccctgcagccctgaatcacttgctgggggtctggaggaggggttcacccttagggctgcttcatggtgggtgggctgactttgtggaaaaatgcccccacttcagccatgtttgtcttatcacggtgcagaaagatcacccaccatctctccttttccttcccagatgctccagaaaacctagatgagcagattaagaaagtgtcccagcagatccttgagaagcgagcctatatctgtgcccaccctctggacaggacatgctgaggcaggggacagtgtcccctgctaccgcccgcccctacccatggcccgttgctggatgactgttactcttttttcagaaggtgttgggattatcacaggttaagccttttgttccccgtctgcacctgaagggttgtcgcctggcctgggagagcctcttccaggttttgacctgcaggcagtgctctctaacaggaccatcacagcttctgaactgagccggagagagagaatggaattgctgacccctggaactggcgggtattctggtcattgaggagacaccatagtggaaactggggcttatgctgctgcctccagggtgtgaggtgggtggggacctgtgtcaggtgtggatagccatttctgctcaaccacacattctctaagaaacagcttgaaagctctgtctgggtcattcatttaaactagaagcagaggcacttaaaacatgtaccaggaaccatttaacaaagaatataaaatgtcacaatctgtgtactgttagcctttgctgtacttgtcacactgttccttagaaccagcctttaatgggtgacagcaggaccctgagaaccaccctttggtgatggcctcgggtcccctttgtcctcaccctgcaaggagggcccagaatgctaaggagcagacacacagtgcaggccacaatcccttggggttatgagcccttagtttttatccttctcaggagatgatggggaggctgtctcagctgatgatgttcccacctagggactttagtttctttacaagaactggcttctactcttgaggagaggatgaatggtatctccaggccagcaggcctttgcatttctccagcctcccttctgctggcacttgaaagattacaccaggtcccagcgtgctcactgtggtgaactttaagctttgatgtggtccttgggtggtctggagctctaaaatgcctattgtggacactcccttgagcacagagaaggcagccgactctttttcctccaagtatattcccaatttactgtgatgctggaaataggcaaggaggagactgggaacttggagagctgagctggctgagtggggctggcctgagcattctgccaggggtttggtaactagtttttaaaatggggaaagtttgtaaatattgtgaccgtgtaaataacctctcagtgaaacctgaagttctgttagtgatagcagggcagcattttgcacaaaatgaagcatgcatacctctggacagaaggctgcttagagtttctttgcacaggagaagtttggggaggggctgtcagacccaccccccttctgtgcagccttctggaagggggcttcactctaggctggtggcgtgtaaggcctcagtcttacatgccaatggagaatggcaagttctccattcatccatctgggttgaaaaggcctagcgaccagttcaagcctctccctctcatctgtagttgctaacttttcttaaacatgttgtgggaagaggagaccccagcaagtgtttcttaagtgatttcaccagtgaaacccccaggagacttttgctgggaaggctggcagtggagctcactaggaagccttcttaccaaggaaaagccttgtgttcttaggctagacagctctcctagctggagcctccttgagagccacagcagtaactgtgggcctgggacatgcccacagagagcaggtctcttcaggcaacctgggagatctagggcctactggggagggagggagccaagtctaggcaaatggagaaagtgacatttcagcaaacttgttagcacttccatggagctgtgatcagttgtccttaggagtcgaggaggagaggaagccatcacgttcacctgacctagttttctgggagaagtttctctggcagaccttgtttttagataggctcatgtctctttctccctgaacaaaggttctggctctgttaaccaagtttgggttctatgttaacctccagatgatcctgagatcaattttcataaacagggataaagaggaagaggacttggagggactggtacagcaagacctacgtttcctgtctctgccttaccccaaagaaagaactgtcagtatctttgccgctggaaggtcccagtgaagcccagagcctctgcccccagctcttggctggacacctagagatcagtcatgggtaatagtgttgaagctcaggaagcctttagacctgtcttccaacttccccactttatagccaagaaaccagacccagggcatgaagggatttgcctcaagtcacacaaatgtcacacttggggctagaatcctggtctgagttccagcccagcattcaatctcttttttcagacccattctgcatcttgcttttcttagcatagaaagtttggttgatagtgtaaacaaaatggataccactgaagatgcagagtggcacagagctcctgcctgcccacggcatcaggaggcccagcttggcaaacccttgcctgttacctgttacaggctttggtgcgggcgaagggagcagctcgaggaaaggtggtggtttcttgtacagatcaaagtccacgtggtgcctgtcccagctccacctgtctcgatccaacacaggctccagtacattagcaaacagggagttttccttccactcctcattcagctctttgatgggtggcagcttgagatcctgaaagctgctttcggtgtcgctctgaagacctgtcacttggaatcccctggctgtgagccaggcctggcgggatttcttctgggctttcttctcctcttccttcaagtccaggggctccaccatggctgagaggtaatcctgtgagtacgtgaatctctttcttggctccttggctatctcttgatacagctccttcttggcaagctctgtagaattcatggtctgggtactatagttgtagacggccttgttggcaggggctgaaattttaatcaccttcgccacggacttcggaggcttcttgctgacctggtaggcttctgtgatatttttctggatgaaactgtgctttttgtctttgttcttcataagcatggcactccgccactgcaggtacttctcctggtgggcgtggatctctaaggtgagggtggagttccgactgtggtagtcctcaagattgggggcaggctgaggtggtagggcaaacagtttctcatctgtgagttcttcttgcgaaaggggcatcccaaactcttggctcaagtcttttatcatagcagaggagggcagcaggtccctcaccgtcacgtcccagagggtggtgctgttatagcagatgtcgtggatcctggctagagcctggaagacccgcctccgctcagtgtctcgcaggaagaacaccgcctgctgcagcagcagctccgtgggctggaagaggtgcacgtggtacaggatggcctccaggtccccatagagccggctgcggaacagcagctgtgagttgtacagcaccttgtatttcctgtgttctgacctgggaatccagctttggtggttctcccacagctgcctcaagccttggtcggccaggccttccaggatgaaaaggtgtgtcttcccgtccagcaggtggaagccagtgagcacatccaggtgctgctgctcctggacccgcacacgcaccttgaaggctgacaggatctgctgcagggtcctgacagggtaggagtccaggccgagggccttagcgttgatcatggtgatgtcctgcagcaggctgtggagcagggagaccttcttaaagtcaaagacgaagatgatgcggccaaactgggagcccccaaggtcaggatcagcagctctggccccggccctcagtggcaccgcgatgtccactcgcaacttgagctgggagtcagcctctaggtagttgcccctgggcattgggccgtgctggtggccatctctggggaccccaagccccacaaccttccttctcctgctgtcctggccgcagtgtgtgggctgaacctcacagctgtggatggggacggccagattcaagtacttgtggccaaggaggaggtcagcaaaactgacctgggcgatgccataagggtaccacatcttgttctgggactcaaaggggttgttctctgtctctctgggagagatgagggcctggaagttgaggtatgaatccagagggtcctccccaaacagcacgggcttctgagaacactcctctgacttgcggtcccggtcgtgaacttccaccaccatgggggggccctccaggtattcccttaggtcactggggtgcagtgccccaaggaagatgacgttgatgtcctggaaataaacgtgggttccatggggctcccccttggtcttgtgaactggagtcttatggaactggtacttgcagtacacaggcatgcacagcctctctagttcctgaatgggtacaggctgtgatggaaggcaggaagcacacttgatctttatggtcaggggatttaaatcctgcttttgctcctcggtcatgatcggaacttctgtttttaaagtcaaaaggcaatctaaaatgttggcagacttctcactgccacgactcacgacagtttgccatccggcaaggagcggcatgacggccagctggatggagaaagcgctctgcttcctggggcctgtcagcgtggggtctgcctcttcttctgccaggggcttcttatgtctcctctggattttccttcttccctctgaatctttccctttaatttgagacctttgtctgtctaatatgtttgttaagctgctaagtgattcactctcaattaattccttgatctccatcatgcttgctcctgccaaagaaatggttggtgttcttgaaacactccattgaatcgtggaagaatcgtccattttgagggacttctcatattcctcactgttcttggaagaagtttcgggctctgcttggtgagaaccttgcaaagactttgggtgtttttctgttttttcttgttttcctggcggatgttcctggttcgactcttctctgacaatgttggtattctcaatgccctgttcagataattttctctgatttaaaaccaaatgtctcacttccatattcacagggaaggccagtgagatggtgaatttgcaggggaccacgtggggcacgtcggagctgaaagtgctggcaggctcagatgaggactcgatgctgctgcacgggcggtcagagtcagactcctgggccctggccttggccttcaggtgttcctccacgtcacactcgctcgtggactggtaaaagctagtgatggaggagatgggctctatgcttgcggggtcctcttcccactcccaggcatgtagcgacatgctgcagagcgcactgctggccgccggcgctcctgctgacatacctcctctgccaagaagctcactgccttccacagcacatccatcattcttcat

SEQ ID NO: 14088 - RNA, 6444 nt, Homo sapiens
  source 1..6444: mol_type = other RNA
gctgggattacaggcatgagccaccgcaccgggcctgccaaggcaattttagattgagcaagtgcagagccctttgcgcaggacccctggcatctgcccagcatgcctggctgtattctcttttttttggagacatagtctcactttgtcacccaggctggctggagtgcagtggcatgatcttggctcactgcaacctccacctcctgggttcaagcaactcctgtgcctcagcctcctgagtagttgggattataggcacgcaccaccatgcccagctaatatttgtatttttagtagaaacaaacagggtttcaccatgttggccaagctggtctccaacccctgacctcaggtgatccgcccaccttggcctcccaaagtgctgggattacaggcatgagccactgtgcccagccctggctgtattcttgaagctgcccggggaaggctcacgaagggaggagcatctggttgtacctgattctggagacagcattttacctgcccctttacccactgtactccatccaaaatgaccctgcagtgccctgcagaggtctcaggccttggcctagagaacagagggctttgctcgtgctccccgctctgtctgcagtgctcttcctcttctatagccactcgaccatatctaggaatgcccagctcagtctacctctgaccctcacagtcctgttgacctgaggttctggatcagtgtccccacaaagcccagtcgtgttgccaagtgatgggtgtaggcgccagcactgtggcacttgctgagagtggcatatgattttttgcaggtcctagccctgggggtagcccagacacccccccagtgctgacaggttatgtgctgtggagggtgctgaaatggtttctcctccagtgggctggaatcacagatgggctgtttacggagcaagtgccggctccaccccatgagatctgggggttagagatgagcaggatgagtcctttgtaactgagaatgaagctgtacccctttctctccctgcagccctgaatcacttgctgggggtctggaggaggggttcacccttagggctgcttcatggtgggtgggctgactttgtggaaaaatgcccccacttcagccatgtttgtcttatcacggtgcagaaagatcacccaccatctctccttttccttcccagatgctccagaaaacctagatgagcagattaagaaagtgtcccagcagatccttgagaagcgagcctatatctgtgcccaccctctggacaggacatgctgaggcaggggacagtgtcccctgctaccgcccgcccctacccatggcccgttgctggatgactgttactcttttttcagaaggtgttgggattatcacaggttaagccttttgttccccgtctgcacctgaagggttgtcgcctggcctgggagagcctcttccaggttttgacctgcaggcagtgctctctaacaggaccatcacagcttctgaactgagccggagagagagaatggaattgctgacccctggaactggcgggtattctggtcattgaggagacaccatagtggaaactggggcttatgctgctgcctccagggtgtgaggtgggtggggacctgtgtcaggtgtggatagccatttctgctcaaccacacattctctaagaaacagcttgaaagctctgtctgggtcattcatttaaactagaagcagaggcacttaaaacatgtaccaggaaccatttaacaaagaatataaaatgtcacaatctgtgtactgttagcctttgctgtacttgtcacactgttccttagaaccagcctttaatgggtgacagcaggaccctgagaaccaccctttggtgatggcctcgggtcccctttgtcctcaccctgcaaggagggcccagaatgctaaggagcagacacacagtgcaggccacaatcccttggggttatgagcccttagtttttatccttctcaggagatgatggggaggctgtctcagctgatgatgttcccacctagggactttagtttctttacaagaactggcttctactcttgaggagaggatgaatggtatctccaggccagcaggcctttgcatttctccagcctcccttctgctggcacttgaaagattacaccaggtcccagcgtgctcactgtggtgaactttaagctttgatgtggtccttgggtggtctggagctctaaaatgcctattgtggacactcccttgagcacagagaaggcagccgactctttttcctccaagtatattcccaatttactgtgatgctggaaataggcaaggaggagactgggaacttggagagctgagctggctgagtggggctggcctgagcattctgccaggggtttggtaactagtttttaaaatggggaaagtttgtaaatattgtgaccgtgtaaataacctctcagtgaaacctgaagttctgttagtgatagcagggcagcattttgcacaaaatgaagcatgcatacctctggacagaaggctgcttagagtttctttgcacaggagaagtttggggaggggctgtcagacccaccccccttctgtgcagccttctggaagggggcttcactctaggctggtggcgtgtaaggcctcagtcttacatgccaatggagaatggcaagttctccattcatccatctgggttgaaaaggcctagcgaccagttcaagcctctccctctcatctgtagttgctaacttttcttaaacatgttgtgggaagaggagaccccagcaagtgtttcttaagtgatttcaccagtgaaacccccaggagacttttgctgggaaggctggcagtggagctcactaggaagccttcttaccaaggaaaagccttgtgttcttaggctagacagctctcctagctggagcctccttgagagccacagcagtaactgtgggcctgggacatgcccacagagagcaggtctcttcaggcaacctgggagatctagggcctactggggagggagggagccaagtctaggcaaatggagaaagtgacatttcagcaaacttgttagcacttccatggagctgtgatcagttgtccttaggagtcgaggaggagaggaagccatcacgttcacctgacctagttttctgggagaagtttctctggcagaccttgtttttagataggctcatgtctctttctccctgaacaaaggttctggctctgttaaccaagtttgggttctatgttaacctccagatgatcctgagatcaattttcataaacagggataaagaggaagaggacttggagggactggtacagcaagacctacgtttcctgtctctgccttaccccaaagaaagaactgtcagtatctttgccgctggaaggtcccagtgaagcccagagcctctgcccccagctcttggctggacacctagagatcagtcatgggtaatagtgttgaagctcaggaagcctttagacctgtcttccaacttccccactttatagccaagaaaccagacccagggcatgaagggatttgcctcaagtcacacaaatgtcacacttggggctagaatcctggtctgagttccagcccagcattcaatctcttttttcagacccattctgcatcttgcttttcttagcatagaaagtttggttgatagtgtaaacaaaatggataccactgaagatgcagagtggcacagagctcctgcctgcccacggcatcaggaggcccagcttggcaaacccttgcctgttacctgttacaggctttggtgcgggcgaagggagcagctcgaggaaaggtggtggtttcttgtacagatcaaagtccacgtggtgcctgtcccagctccacctgtctcgatccaacacaggctccagtacattagcaaacagggagttttccttccactcctcattcagctctttgatgggtggcagcttgagatcctgaaagctgctttcggtgtcgctctgaagacctgtcacttggaatcccctggctgtgagccaggcctggcgggatttcttctgggctttcttctcctcttccttcaagtccaggggctccaccatggctgagaggtaatcctgtgagtacgtgaatctctttcttggctccttggctatctcttgatacagctccttcttggcaagctctgtagaattcatggtctgggtactatagttgtagacggccttgttggcaggggctgaaattttaatcaccttcgccacggacttcggaggcttcttgctgacctggtaggcttctgtgatatttttctggatgaaactgtgctttttgtctttgttcttcataagcatggcactccgccactgcaggtacttctcctggtgggcgtggatctctaaggtgagggtggagttccgactgtggtagtcctcaagattgggggcaggctgaggtggtagggcaaacagtttctcatctgtgagttcttcttgcgaaaggggcatcccaaactcttggctcaagtcttttatcatagcagaggagggcagcaggtccctcaccgtcacgtcccagagggtggtgctgttatagcagatgtcgtggatcctggctagagcctggaagacccgcctccgctcagtgtctcgcaggaagaacaccgcctgctgcagcagcagctccgtgggctggaagaggtgcacgtggtacaggatggcctccaggtccccatagagccggctgcggaacagcagctgtgagttgtacagcaccttgtatttcctgtgttctgacctgggaatccagctttggtggttctcccacagctgcctcaagccttggtcggccaggccttccaggatgaaaaggtgtgtcttcccgtccagcaggtggaagccagtgagcacatccaggtgctgctgctcctggacccgcacacgcaccttgaaggctgacaggatctgctgcagggtcctgacagggtaggagtccaggccgagggccttagcgttgatcatggtgatgtcctgcagcaggctgtggagcagggagaccttcttaaagtcaaagacgaagatgatgcggccaaactgggagcccccaaggtcaggatcagcagctctggccccggccctcagtggcaccgcgatgtccactcgcaacttgagctgggagtcagcctctaggtagttgcccctgggcattgggccgtgctggtggccatctctggggaccccaagccccacaaccttccttctcctgctgtcctggccgcagtgtgtgggctgaacctcacagctgtggatggggacggccagattcaagtacttgtggccaaggaggaggtcagcaaaactgacctgggcgatgccataagggtaccacatcttgttctgggactcaaaggggttgttctctgtctctctgggagagatgagggcctggaagttgaggtatgaatccagagggtcctccccaaacagcacgggcttctgagaacactcctctgacttgcggtcccggtcgtgaacttccaccaccatgggggggccctccaggtattcccttaggtcactggggtgcagtgccccaaggaagatgacgttgatgtcctggaaataaacgtgggttccatggggctcccccttggtcttgtgaactggagtcttatggaactggtacttgcagtacacaggcatgcacagcctctctagttcctgaatgggtacaggctgtgatggaaggcaggaagcacacttgatctttatggtcaggggatttaaatcctgcttttgctcctcggtcatgatcggaacttctgtttttaaagtcaaaaggcaatctaaaatgttggcagacttctcactgccacgactcacgacagtttgccatccggcaaggagcggcatgacggccagctggatggagaaagcgctctgcttcctggggcctgtcagcgtggggtctgcctcttcttctgccaggggcttcttatgtctcctctggattttccttcttccctctgaatctttccctttaatttgagacctttgtctgtctaatatgtttgttaagctgctaagtgattcactctcaattaattccttgatctccatcatgcttgctcctgccaaagaaatggttggtgttcttgaaacactccattgaatcgtggaagaatcgtccattttgagggacttctcatattcctcactgttcttggaagaagtttcgggctctgcttggtgagaaccttgcaaagactttgggtgtttttctgttttttcttgttttcctggcggatgttcctggttcgactcttctctgacaatgttggtattctcaatgccctgttcagataattttctctgatttaaaaccaaatgtctcacttccgtggtcccagctactcaggaggctgaggcagga

SEQ ID NO: 14089 - RNA, 12487 nt, Homo sapiens
  source 1..12487: mol_type = other RNA
gctgggattacaggcatgagccaccgcaccgggcctgccaaggcaattttagattgagcaagtgcagagccctttgcgcaggacccctggcatctgcccagcatgcctggctgtattctcttttttttggagacatagtctcactttgtcacccaggctggctggagtgcagtggcatgatcttggctcactgcaacctccacctcctgggttcaagcaactcctgtgcctcagcctcctgagtagttgggattataggcacgcaccaccatgcccagctaatatttgtatttttagtagaaacaaacagggtttcaccatgttggccaagctggtctccaacccctgacctcaggtgatccgcccaccttggcctcccaaagtgctgggattacaggcatgagccactgtgcccagccctggctgtattcttgaagctgcccggggaaggctcacgaagggaggagcatctggttgtacctgattctggagacagcattttacctgcccctttacccactgtactccatccaaaatgaccctgcagtgccctgcagaggtctcaggccttggcctagagaacagagggctttgctcgtgctccccgctctgtctgcagtgctcttcctcttctatagccactcgaccatatctaggaatgcccagctcagtctacctctgaccctcacagtcctgttgacctgaggttctggatcagtgtccccacaaagcccagtcgtgttgccaagtgatgggtgtaggcgccagcactgtggcacttgctgagagtggcatatgattttttgcaggtcctagccctgggggtagcccagacacccccccagtgctgacaggttatgtgctgtggagggtgctgaaatggtttctcctccagtgggctggaatcacagatgggctgtttacggagcaagtgccggctccaccccatgagatctgggggttagagatgagcaggatgagtcctttgtaactgagaatgaagctgtacccctttctctccctgcagccctgaatcacttgctgggggtctggaggaggggttcacccttagggctgcttcatggtgggtgggctgactttgtggaaaaatgcccccacttcagccatgtttgtcttatcacggtgcagaaagatcacccaccatctctccttttccttcccagatgctccagaaaacctagatgagcagattaagaaagtgtcccagcagatccttgagaagcgagcctatatctgtgcccaccctctggacaggacatgctgaggcaggggacagtgtcccctgctaccgcccgcccctacccatggcccgttgctggatgactgttactcttttttcagaaggtgttgggattatcacaggttaagccttttgttccccgtctgcacctgaagggttgtcgcctggcctgggagagcctcttccaggttttgacctgcaggcagtgctctctaacaggaccatcacagcttctgaactgagccggagagagagaatggaattgctgacccctggaactggcgggtattctggtcattgaggagacaccatagtggaaactggggcttatgctgctgcctccagggtgtgaggtgggtggggacctgtgtcaggtgtggatagccatttctgctcaaccacacattctctaagaaacagcttgaaagctctgtctgggtcattcatttaaactagaagcagaggcacttaaaacatgtaccaggaaccatttaacaaagaatataaaatgtcacaatctgtgtactgttagcctttgctgtacttgtcacactgttccttagaaccagcctttaatgggtgacagcaggaccctgagaaccaccctttggtgatggcctcgggtcccctttgtcctcaccctgcaaggagggcccagaatgctaaggagcagacacacagtgcaggccacaatcccttggggttatgagcccttagtttttatccttctcaggagatgatggggaggctgtctcagctgatgatgttcccacctagggactttagtttctttacaagaactggcttctactcttgaggagaggatgaatggtatctccaggccagcaggcctttgcatttctccagcctcccttctgctggcacttgaaagattacaccaggtcccagcgtgctcactgtggtgaactttaagctttgatgtggtccttgggtggtctggagctctaaaatgcctattgtggacactcccttgagcacagagaaggcagccgactctttttcctccaagtatattcccaatttactgtgatgctggaaataggcaaggaggagactgggaacttggagagctgagctggctgagtggggctggcctgagcattctgccaggggtttggtaactagtttttaaaatggggaaagtttgtaaatattgtgaccgtgtaaataacctctcagtgaaacctgaagttctgttagtgatagcagggcagcattttgcacaaaatgaagcatgcatacctctggacagaaggctgcttagagtttctttgcacaggagaagtttggggaggggctgtcagacccaccccccttctgtgcagccttctggaagggggcttcactctaggctggtggcgtgtaaggcctcagtcttacatgccaatggagaatggcaagttctccattcatccatctgggttgaaaaggcctagcgaccagttcaagcctctccctctcatctgtagttgctaacttttcttaaacatgttgtgggaagaggagaccccagcaagtgtttcttaagtgatttcaccagtgaaacccccaggagacttttgctgggaaggctggcagtggagctcactaggaagccttcttaccaaggaaaagccttgtgttcttaggctagacagctctcctagctggagcctccttgagagccacagcagtaactgtgggcctgggacatgcccacagagagcaggtctcttcaggcaacctgggagatctagggcctactggggagggagggagccaagtctaggcaaatggagaaagtgacatttcagcaaacttgttagcacttccatggagctgtgatcagttgtccttaggagtcgaggaggagaggaagccatcacgttcacctgacctagttttctgggagaagtttctctggcagaccttgtttttagataggctcatgtctctttctccctgaacaaaggttctggctctgttaaccaagtttgggttctatgttaacctccagatgatcctgagatcaattttcataaacagggataaagaggaagaggacttggagggactggtacagcaagacctacgtttcctgtctctgccttaccccaaagaaagaactgtcagtatctttgccgctggaaggtcccagtgaagcccagagcctctgcccccagctcttggctggacacctagagatcagtcatgggtaatagtgttgaagctcaggaagcctttagacctgtcttccaacttccccactttatagccaagaaaccagacccagggcatgaagggatttgcctcaagtcacacaaatgtcacacttggggctagaatcctggtctgagttccagcccagcattcaatctcttttttcagacccattctgcatcttgcttttcttagcatagaaagtttggttgatagtgtaaacaaaatggataccactgaagatgcagagtggcacagagctcctgcctgcccacggcatcaggaggcccagcttggcaaacccttgcctgttacctgttacaggctttggtgcgggcgaagggagcagctcgaggaaaggtggtggtttcttgtacagatcaaagtccacgtggtgcctgtcccagctccacctgtctcgatccaacacaggctccagtacattagcaaacagggagttttccttccactcctcattcagctctttgatgggtggcagcttgagatcctgaaagctgctttcggtgtcgctctgaagacctgtcacttggaatcccctggctgtgagccaggcctggcgggatttcttctgggctttcttctcctcttccttcaagtccaggggctccaccatggctgagaggtaatcctgtgagtacgtgaatctctttcttggctccttggctatctcttgatacagctccttcttggcaagctctgtagaattcatggtctgggtactatagttgtagacggccttgttggcaggggctgaaattttaatcaccttcgccacggacttcggaggcttcttgctgacctggtaggcttctgtgatatttttctggatgaaactgtgctttttgtctttgttcttcataagcatggcactccgccactgcaggtacttctcctggtgggcgtggatctctaaggtgagggtggagttccgactgtggtagtcctcaagattgggggcaggctgaggtggtagggcaaacagtttctcatctgtgagttcttcttgcgaaaggggcatcccaaactcttggctcaagtcttttatcatagcagaggagggcagcaggtccctcaccgtcacgtcccagagggtggtgctgttatagcagatgtcgtggatcctggctagagcctggaagacccgcctccgctcagtgtctcgcaggaagaacaccgcctgctgcagcagcagctccgtgggctggaagaggtgcacgtggtacaggatggcctccaggtccccatagagccggctgcggaacagcagctgtgagttgtacagcaccttgtatttcctgtgttctgacctgggaatccagctttggtggttctcccacagctgcctcaagccttggtcggccaggccttccaggatgaaaaggtgtgtcttcccgtccagcaggtggaagccagtgagcacatccaggtgctgctgctcctggacccgcacacgcaccttgaaggctgacaggatctgctgcagggtcctgacagggtaggagtccaggccgagggccttagcgttgatcatggtgatgtcctgcagcaggctgtggagcagggagaccttcttaaagtcaaagacgaagatgatgcggccaaactgggagcccccaaggtcaggatcagcagctctggccccggccctcagtggcaccgcgatgtccactcgcaacttgagctgggagtcagcctctaggtagttgcccctgggcattgggccgtgctggtggccatctctggggaccccaagccccacaaccttccttctcctgctgtcctggccgcagtgtgtgggctgaacctcacagctgtggatggggacggccagattcaagtacttgtggccaaggaggaggtcagcaaaactgacctgggcgatgccataagggtaccacatcttgttctgggactcaaaggggttgttctctgtctctctgggagagatgagggcctggaagttgaggtatgaatccagagggtcctccccaaacagcacgggcttctgagaacactcctctgacttgcggtcccggtcgtgaacttccaccaccatgggggggccctccaggtattcccttaggtcactggggtgcagtgccccaaggaagatgacgttgatgtcctggaaataaacgtgggttccatggggctcccccttggtcttgtgaactggagtcttatggaactggtacttgcagtacacaggcatgcacagcctctctagttcctgaatgggtacaggctgtgatggaaggcaggaagcacacttgatctttatggtcaggggatttaaatcctgcttttgctcctcggtcatgatcggaacttctgtttttaaagtcaaaaggcaatctaaaatgttggcagacttctcactgccacgactcacgacagtttgccatccggcaaggagcggcatgacggccagctggatggagaaagcgctctgcttcctggggcctgtcagcgtggggtctgcctcttcttctgccaggggcttcttatgtctcctctggattttccttcttccctctgaatctttccctttaatttgagacctttgtctgtctaatatgtttgttaagctgctaagtgattcactctcaattaattccttgatctccatcatgcttgctcctgccaaagaaatggttggtgttcttgaaacactccattgaatcgtggaagaatcgtccattttgagggacttctcatattcctcactgttcttggaagaagtttcgggctctgcttggtgagaaccttgcaaagactttgggtgtttttctgttttttcttgttttcctggcggatgttcctggttcgactcttctctgacaatgttggtattctcaatgccctgttcagataattttctctgatttaaaaccaaatgtctcacttctgacttatgaaaagctcccacgtcgtctgtgaagccggcagtctttaatcggtaatatctgacttttcttgacatcttgtctttagtgttccagagcctcaaggtgattttgtggaaatttattttctttaataattcctttgtcacagtgatattaaaagtctgctcccacgacacccaggctttgtcaccttcgtgccacggcttcacagtccatattcacagggaaggccagtgagatggtgaatttgcaggggaccacgtggggcacgtcggagctgaaagtgctggcaggctcagatgaggactcgatgctgctgcacgggcggtcagagtcagactcctgggccctggccttggccttcaggtgttcctccacgtcacactcgctcgtggactggtaaaagctagtgatggaggagatgggctctatgcttgcggggtcctcttcccactcccaggcatgtagcgacatgctgcagagcgcactgctggccgccggcgctcctgcgagcggatgcgctgggcggcagcggggagttggaccgcggcggcaactcccgtaccggatccacagccacctgggcgaagagactccaagactgagaggagcgtccgccggtgcagggagggccgcaggcccagccactcagctacgtttggcggttgctaggagacgcgagggcgtgcggcctgggggcggggctccgcggggcggggctttccccctcagccactgcgcgcagtttgtcaaatggctacatccaggttcagaaaccagctgccttcattccttcactcatgcattcactcattaaggagtttctactcggaacgtcagcacctactataagcctggtccttgcccgtacgatgggaggtaggggttgatggctccttcctccccctccatcagctcccacctcccattctttaataaaagcaaaggaagctgtgggctctgcaaactccagacctccccacgatccctctcattagattctctgcttctgtcgccgatgtccttaaaaaccagacctccccacgatccctctcattagattctctgcttctgtcgctgatgtccttaaaatagcatgagaattcttgttagtgatcatgagcgccaactcagagatcagaaaacaaagcttagagaggtgaagcgattcgcccgaggtcacacagcaagtagggcgcagcactgtgttgaaatccggactgcctgactccaaagcctccgctcgtctgctaaaccacccaagctgagagccctggctgcggctcctaatgtagaggacctcagcacagcaagcggctgggacagagggctggggtaggcctcatggaggaagtgagcaacgccaaatctggggggtgactaggcagaggcggtgaaagcaagagaaagcatcccaggtagaggaacagcatatgcaaaggcccatagaggtgaaagggcatggcaagtttcaggaatgggtggcgaggctgtagcagtgtgcagggcccatggtacatagccccacagggcaggttagggcacaggactatgggcaatggggagccaaggcaggtcttctgttgagggagggcaccctgctccggcagtcagtttgttcaagagaatgggagctgaggctacacacaagcttggctattaagaaaactttagctgagttgagctatgacctactttgtgtcaaagagcaaaactgtggcgcagctggggctgagacccaagtcctgagcctcccagtgcatgcctccccagaccgctctcagggcatgggacagcccctttaatactgggtgctccaatactcctcgggttcagtctgaaaaacagcctcaagtacagctgttagggaagacaccaaatggcagtgggccctgtgaggagtgggttcaaactcttagcacgagaacggcaaccaccttgcccacaccccacctgcagcagcctggagactgctgtctgtatgccaggaagtgctcaggagacacatgaagggctggaagaatacaaagctactcagatacaccagcccccaaaagggccctttaacaagggcagttcaacactaccaccactcttggacagacatcaggcctcctgctccccaggtcctacccactggcctgaggctggtttccctccaaaggttcctagatcacatcaccacctaggacagaagccaatctcttcccaagctcaatagtgagaggccagaggtcttggaccaagggccaatgtgccatcctggatgtgcactggaaacacctacatgtcaaaaatacaattctgaggcttcattaaagacctgtggaagtgactctccaggggtggagcttagaaaccagtggcagattgtattttccaaagacagccacctcaaaagatcccctcccacataatcttccggcaggcattgtgaggttcacattcctcccacccagttggggggtctagtctccttctctggaaactgggcagacctctgtgactggctcagtcaaaagagtgcagaggaaatgacactatgtgatttctgaggccaggtcatataaattccatctacctctgccctgttcttttgaggtatagtattcatgctaggaatccagctagcatgttgtgaggaagcccaagcagccatgtgaaatggccacatgaaactgttgtgactgacggttcccagccaattgcagcctcaacccccagacatatgagagtgcaagacttcaaatgatcccagccctcagtctttgagccaccctggctgacattgaggaacagaaacaagctgtctccatcatgagaaattgtagatttataagcaaattgttgctctcttaaaccactaagttttggggtgatttgttgtgcaataaataataggaacgggagccatatttttaaattaccaccaagattgtattgcacaaccagaatatggaaccactgccctgagagagatggtgtctgggtcaagacctagggcatcacaggatgaagtgagggcaaaggtgtgctacccactactcaggtatgagacagtggtgggtctacaaccctacctcagtgaagatggcttcagggctggcagatcagaagcaaaggaaggggggcttctgtttcagttatctgttactgagtaaaaaccatccccaaacttaatggtgtcaaacaaacacttgttatttctcaccactccatgcatcagctgagtagttctctgctggcctcgcctgggctcactccctatgctgtgctcagctggaggaccaacatggctggaagctgccagaagtcctcacttgcatgtctggcagttgctgctggctcttcgtgggcccgctggttcccctccatgggttcccccgcccccagtggtacaccagcttccttctatgtggtgcctcatctcctcatagcccggcctggcttcctcagatggcattctcagagcagggatcccagagggcaaagaagaagttgcaaggcctcttgggacctaggcgtggaaccagcaccatgtcactctgctacatgccattaaccaaagcaagtcatgaggctggccccacttcaaggggatgaagacatggactgtacatctggtaagcagagggacaagcatccaggggcaggaggtgttcaaggtcactgaacaatccatcccttcatccttactctgccgggtggagggttcccaagctcccacaggctatgtagaggccttcctgaagctatcccaagactctggcagctggaagcatattgggaatcagctacatacaccttcttcttgccccttccccatttttaacagctttattgaagtattttttatttaataaaatccatccatttcaagcgtagaattcaatgattttcagtaactttacctagtgctgtaatcatcatcataaattcattttagaacattttcatccccctaataagacttcatgcacatttataattaatctctgttccaactcccagtcctaggcaaccatatctactttgtttctaaaaattggccttttctagacatttcctataaattgagtcagacactgtgttctggctttgtgactggtttctttcacctaccgttatgtttccaaggtttatttatgttgaggcatgtgtcagtatttcattccttttcatgactgaataatattctattgtatggacagaccacagtttgcctatccattcatcagttaatgggcatttggcttgggcatttagacatttatgaacaacgttgctatgaacattcccacacaagtctttgtgtggatgtgttttcatctctcttgggtcgatatctaggagtggaagagttgggtcgtatggtcattttgtgattaacttcttgagaaactgccaaactatcttccacaggggctgcatcattttgtgttcccatcaacaacatgaagtttcctgtttctccaaattcttgacaagatttattgcctgttttattcactacagctattctcatgagtataatatagtatttcatcatagttttcatgtgcatttccctaacaagaatactgagattgttttatgcacatgttggctatttatacaacttctttggtgaaatgtctgtttgtatcttcacccactttttgattggattgtttgtcttcttgttactgagttgttaagagttcattgtaaattcggaatataagtcctttactgggcatatgttttacaaatattttctcctagtctcttgttcgtcatattttcttaatagtgtcttttgaagtgcaaatgttttgaactttgatgaaggtccgattcatcatttttttcttttttggatcatgcatttggtgtcgtatctaagaaatctttgactaacaacaggcctatttttaatagaagtaaagcttggtgtctgaacactaagcaaatctactaaccaagacccctaaaaacccaaaagctttatgacactgaaaataatggcccaaggacattcccagacagttctgggctctggatagaacaacacaagtttccaaaaaacaggctgataataccacaagcttataaaatatgtatactccttggcccagtaataaatcactcaagatatggcacaaactgttcacagtatggtttttgcggagaaaagctgaaaaccacctcagtgggcatctgtgggggatgacaaagcaccttatagttcatccccagggagcacagagcagcctctggagcagtgtctgcaaagaaaccacagccaagctgtttacaaagctcagttcctgtgcaaagaaagatcccaatggcgccctttccactgtgcttttcatgtcaagttgaatgagctacgatttgcacactgtaaaattcagatgtacacagtcatgcaaccactacaccatgaagatagagtatttcaatcactccaaaaagttctttcatgcccaaatacatagaaaagtctggaaataaatacatcagaaatacacagtgatcctctcttggtggcagaatggtggatgatttttgctttttagcattttcccggacctttaaaagacactttaaacaatatactatttgaaatggctcaaacaatactgaactgacttcagaaaatcatttctttgccacagccctgactctctcccacacagacacacgcccatccccccagctcatacaaaagaacgcaaggagacctctgagtttgctcactttgaaccttaaacaaaaaccttgtggatgcaaccagaattatttcagaggtgcctggtaacaccgcagggcagacagacaggcctgacagcaaaccattatcaacccttacttccctgagctgtaggggagtggaggccggcaacggctcccagcaagacatttaaaagctttcttttcaatattgactggcccaggaaagctactgttcaaaggattccttcaccagctgcagggatggggggtggggagggtgttgcactcttgcctgggctaccagctcttagggctgacatgaaataaaatcaggttctttttttttttttttttt

SEQ ID NO: 14090 - RNA, 6667 nt, Homo sapiens
  source 1..6667: mol_type = other RNA
gctgggattacaggcatgagccaccgcaccgggcctgccaaggcaattttagattgagcaagtgcagagccctttgcgcaggacccctggcatctgcccagcatgcctggctgtattctcttttttttggagacatagtctcactttgtcacccaggctggctggagtgcagtggcatgatcttggctcactgcaacctccacctcctgggttcaagcaactcctgtgcctcagcctcctgagtagttgggattataggcacgcaccaccatgcccagctaatatttgtatttttagtagaaacaaacagggtttcaccatgttggccaagctggtctccaacccctgacctcaggtgatccgcccaccttggcctcccaaagtgctgggattacaggcatgagccactgtgcccagccctggctgtattcttgaagctgcccggggaaggctcacgaagggaggagcatctggttgtacctgattctggagacagcattttacctgcccctttacccactgtactccatccaaaatgaccctgcagtgccctgcagaggtctcaggccttggcctagagaacagagggctttgctcgtgctccccgctctgtctgcagtgctcttcctcttctatagccactcgaccatatctaggaatgcccagctcagtctacctctgaccctcacagtcctgttgacctgaggttctggatcagtgtccccacaaagcccagtcgtgttgccaagtgatgggtgtaggcgccagcactgtggcacttgctgagagtggcatatgattttttgcaggtcctagccctgggggtagcccagacacccccccagtgctgacaggttatgtgctgtggagggtgctgaaatggtttctcctccagtgggctggaatcacagatgggctgtttacggagcaagtgccggctccaccccatgagatctgggggttagagatgagcaggatgagtcctttgtaactgagaatgaagctgtacccctttctctccctgcagccctgaatcacttgctgggggtctggaggaggggttcacccttagggctgcttcatggtgggtgggctgactttgtggaaaaatgcccccacttcagccatgtttgtcttatcacggtgcagaaagatcacccaccatctctccttttccttcccagatgctccagaaaacctagatgagcagattaagaaagtgtcccagcagatccttgagaagcgagcctatatctgtgcccaccctctggacaggacatgctgaggcaggggacagtgtcccctgctaccgcccgcccctacccatggcccgttgctggatgactgttactcttttttcagaaggtgttgggattatcacaggttaagccttttgttccccgtctgcacctgaagggttgtcgcctggcctgggagagcctcttccaggttttgacctgcaggcagtgctctctaacaggaccatcacagcttctgaactgagccggagagagagaatggaattgctgacccctggaactggcgggtattctggtcattgaggagacaccatagtggaaactggggcttatgctgctgcctccagggtgtgaggtgggtggggacctgtgtcaggtgtggatagccatttctgctcaaccacacattctctaagaaacagcttgaaagctctgtctgggtcattcatttaaactagaagcagaggcacttaaaacatgtaccaggaaccatttaacaaagaatataaaatgtcacaatctgtgtactgttagcctttgctgtacttgtcacactgttccttagaaccagcctttaatgggtgacagcaggaccctgagaaccaccctttggtgatggcctcgggtcccctttgtcctcaccctgcaaggagggcccagaatgctaaggagcagacacacagtgcaggccacaatcccttggggttatgagcccttagtttttatccttctcaggagatgatggggaggctgtctcagctgatgatgttcccacctagggactttagtttctttacaagaactggcttctactcttgaggagaggatgaatggtatctccaggccagcaggcctttgcatttctccagcctcccttctgctggcacttgaaagattacaccaggtcccagcgtgctcactgtggtgaactttaagctttgatgtggtccttgggtggtctggagctctaaaatgcctattgtggacactcccttgagcacagagaaggcagccgactctttttcctccaagtatattcccaatttactgtgatgctggaaataggcaaggaggagactgggaacttggagagctgagctggctgagtggggctggcctgagcattctgccaggggtttggtaactagtttttaaaatggggaaagtttgtaaatattgtgaccgtgtaaataacctctcagtgaaacctgaagttctgttagtgatagcagggcagcattttgcacaaaatgaagcatgcatacctctggacagaaggctgcttagagtttctttgcacaggagaagtttggggaggggctgtcagacccaccccccttctgtgcagccttctggaagggggcttcactctaggctggtggcgtgtaaggcctcagtcttacatgccaatggagaatggcaagttctccattcatccatctgggttgaaaaggcctagcgaccagttcaagcctctccctctcatctgtagttgctaacttttcttaaacatgttgtgggaagaggagaccccagcaagtgtttcttaagtgatttcaccagtgaaacccccaggagacttttgctgggaaggctggcagtggagctcactaggaagccttcttaccaaggaaaagccttgtgttcttaggctagacagctctcctagctggagcctccttgagagccacagcagtaactgtgggcctgggacatgcccacagagagcaggtctcttcaggcaacctgggagatctagggcctactggggagggagggagccaagtctaggcaaatggagaaagtgacatttcagcaaacttgttagcacttccatggagctgtgatcagttgtccttaggagtcgaggaggagaggaagccatcacgttcacctgacctagttttctgggagaagtttctctggcagaccttgtttttagataggctcatgtctctttctccctgaacaaaggttctggctctgttaaccaagtttgggttctatgttaacctccagatgatcctgagatcaattttcataaacagggataaagaggaagaggacttggagggactggtacagcaagacctacgtttcctgtctctgccttaccccaaagaaagaactgtcagtatctttgccgctggaaggtcccagtgaagcccagagcctctgcccccagctcttggctggacacctagagatcagtcatgggtaatagtgttgaagctcaggaagcctttagacctgtcttccaacttccccactttatagccaagaaaccagacccagggcatgaagggatttgcctcaagtcacacaaatgtcacacttggggctagaatcctggtctgagttccagcccagcattcaatctcttttttcagacccattctgcatcttgcttttcttagcatagaaagtttggttgatagtgtaaacaaaatggataccactgaagatgcagagtggcacagagctcctgcctgcccacggcatcaggaggcccagcttggcaaacccttgcctgttacctgttacaggctttggtgcgggcgaagggagcagctcgaggaaaggtggtggtttcttgtacagatcaaagtccacgtggtgcctgtcccagctccacctgtctcgatccaacacaggctccagtacattagcaaacagggagttttccttccactcctcattcagctctttgatgggtggcagcttgagatcctgaaagctgctttcggtgtcgctctgaagacctgtcacttggaatcccctggctgtgagccaggcctggcgggatttcttctgggctttcttctcctcttccttcaagtccaggggctccaccatggctgagaggtaatcctgtgagtacgtgaatctctttcttggctccttggctatctcttgatacagctccttcttggcaagctctgtagaattcatggtctgggtactatagttgtagacggccttgttggcaggggctgaaattttaatcaccttcgccacggacttcggaggcttcttgctgacctggtaggcttctgtgatatttttctggatgaaactgtgctttttgtctttgttcttcataagcatggcactccgccactgcaggtacttctcctggtgggcgtggatctctaaggtgagggtggagttccgactgtggtagtcctcaagattgggggcaggctgaggtggtagggcaaacagtttctcatctgtgagttcttcttgcgaaaggggcatcccaaactcttggctcaagtcttttatcatagcagaggagggcagcaggtccctcaccgtcacgtcccagagggtggtgctgttatagcagatgtcgtggatcctggctagagcctggaagacccgcctccgctcagtgtctcgcaggaagaacaccgcctgctgcagcagcagctccgtgggctggaagaggtgcacgtggtacaggatggcctccaggtccccatagagccggctgcggaacagcagctgtgagttgtacagcaccttgtatttcctgtgttctgacctgggaatccagctttggtggttctcccacagctgcctcaagccttggtcggccaggccttccaggatgaaaaggtgtgtcttcccgtccagcaggtggaagccagtgagcacatccaggtgctgctgctcctggacccgcacacgcaccttgaaggctgacaggatctgctgcagggtcctgacagggtaggagtccaggccgagggccttagcgttgatcatggtgatgtcctgcagcaggctgtggagcagggagaccttcttaaagtcaaagacgaagatgatgcggccaaactgggagcccccaaggtcaggatcagcagctctggccccggccctcagtggcaccgcgatgtccactcgcaacttgagctgggagtcagcctctaggtagttgcccctgggcattgggccgtgctggtggccatctctggggaccccaagccccacaaccttccttctcctgctgtcctggccgcagtgtgtgggctgaacctcacagctgtggatggggacggccagattcaagtacttgtggccaaggaggaggtcagcaaaactgacctgggcgatgccataagggtaccacatcttgttctgggactcaaaggggttgttctctgtctctctgggagagatgagggcctggaagttgaggtatgaatccagagggtcctccccaaacagcacgggcttctgagaacactcctctgacttgcggtcccggtcgtgaacttccaccaccatgggggggccctccaggtattcccttaggtcactggggtgcagtgccccaaggaagatgacgttgatgtcctggaaataaacgtgggttccatggggctcccccttggtcttgtgaactggagtcttatggaactggtacttgcagtacacaggcatgcacagcctctctagttcctgaatgggtacaggctgtgatggaaggcaggaagcacacttgatctttatggtcaggggatttaaatcctgcttttgctcctcggtcatgatcggaacttctgtttttaaagtcaaaaggcaatctaaaatgttggcagacttctcactgccacgactcacgacagtttgccatccggcaaggagcggcatgacggccagctggatggagaaagcgctctgcttcctggggcctgtcagcgtggggtctgcctcttcttctgccaggggcttcttatgtctcctctggattttccttcttccctctgaatctttccctttaatttgagacctttgtctgtctaatatgtttgttaagctgctaagtgattcactctcaattaattccttgatctccatcatgcttgctcctgccaaagaaatggttggtgttcttgaaacactccattgaatcgtggaagaatcgtccattttgagggacttctcatattcctcactgttcttggaagaagtttcgggctctgcttggtgagaaccttgcaaagactttgggtgtttttctgttttttcttgttttcctggcggatgttcctggttcgactcttctctgacaatgttggtattctcaatgccctgttcagataattttctctgatttaaaaccaaatgtctcacttctgacttatgaaaagctcccacgtcgtctgtgaagccggcagtctttaatcggtaatatctgacttttcttgacatcttgtctttagtgttccagagcctcaaggtgattttgtggaaatttattttctttaataattcctttgtcacagtgatattaaaagtctgctcccacgacacccaggctttgtcaccttcgtgccacggcttcacagtctgcgagcggatgcgctgggcggcagcggggagttggaccgcgg

SEQ ID NO: 14091 - RNA, 6661 nt, Homo sapiens
  source 1..6661: mol_type = other RNA
gctgggattacaggcatgagccaccgcaccgggcctgccaaggcaattttagattgagcaagtgcagagccctttgcgcaggacccctggcatctgcccagcatgcctggctgtattctcttttttttggagacatagtctcactttgtcacccaggctggctggagtgcagtggcatgatcttggctcactgcaacctccacctcctgggttcaagcaactcctgtgcctcagcctcctgagtagttgggattataggcacgcaccaccatgcccagctaatatttgtatttttagtagaaacaaacagggtttcaccatgttggccaagctggtctccaacccctgacctcaggtgatccgcccaccttggcctcccaaagtgctgggattacaggcatgagccactgtgcccagccctggctgtattcttgaagctgcccggggaaggctcacgaagggaggagcatctggttgtacctgattctggagacagcattttacctgcccctttacccactgtactccatccaaaatgaccctgcagtgccctgcagaggtctcaggccttggcctagagaacagagggctttgctcgtgctccccgctctgtctgcagtgctcttcctcttctatagccactcgaccatatctaggaatgcccagctcagtctacctctgaccctcacagtcctgttgacctgaggttctggatcagtgtccccacaaagcccagtcgtgttgccaagtgatgggtgtaggcgccagcactgtggcacttgctgagagtggcatatgattttttgcaggtcctagccctgggggtagcccagacacccccccagtgctgacaggttatgtgctgtggagggtgctgaaatggtttctcctccagtgggctggaatcacagatgggctgtttacggagcaagtgccggctccaccccatgagatctgggggttagagatgagcaggatgagtcctttgtaactgagaatgaagctgtacccctttctctccctgcagccctgaatcacttgctgggggtctggaggaggggttcacccttagggctgcttcatggtgggtgggctgactttgtggaaaaatgcccccacttcagccatgtttgtcttatcacggtgcagaaagatcacccaccatctctccttttccttcccagatgctccagaaaacctagatgagcagattaagaaagtgtcccagcagatccttgagaagcgagcctatatctgtgcccaccctctggacaggacatgctgaggcaggggacagtgtcccctgctaccgcccgcccctacccatggcccgttgctggatgactgttactcttttttcagaaggtgttgggattatcacaggttaagccttttgttccccgtctgcacctgaagggttgtcgcctggcctgggagagcctcttccaggttttgacctgcaggcagtgctctctaacaggaccatcacagcttctgaactgagccggagagagagaatggaattgctgacccctggaactggcgggtattctggtcattgaggagacaccatagtggaaactggggcttatgctgctgcctccagggtgtgaggtgggtggggacctgtgtcaggtgtggatagccatttctgctcaaccacacattctctaagaaacagcttgaaagctctgtctgggtcattcatttaaactagaagcagaggcacttaaaacatgtaccaggaaccatttaacaaagaatataaaatgtcacaatctgtgtactgttagcctttgctgtacttgtcacactgttccttagaaccagcctttaatgggtgacagcaggaccctgagaaccaccctttggtgatggcctcgggtcccctttgtcctcaccctgcaaggagggcccagaatgctaaggagcagacacacagtgcaggccacaatcccttggggttatgagcccttagtttttatccttctcaggagatgatggggaggctgtctcagctgatgatgttcccacctagggactttagtttctttacaagaactggcttctactcttgaggagaggatgaatggtatctccaggccagcaggcctttgcatttctccagcctcccttctgctggcacttgaaagattacaccaggtcccagcgtgctcactgtggtgaactttaagctttgatgtggtccttgggtggtctggagctctaaaatgcctattgtggacactcccttgagcacagagaaggcagccgactctttttcctccaagtatattcccaatttactgtgatgctggaaataggcaaggaggagactgggaacttggagagctgagctggctgagtggggctggcctgagcattctgccaggggtttggtaactagtttttaaaatggggaaagtttgtaaatattgtgaccgtgtaaataacctctcagtgaaacctgaagttctgttagtgatagcagggcagcattttgcacaaaatgaagcatgcatacctctggacagaaggctgcttagagtttctttgcacaggagaagtttggggaggggctgtcagacccaccccccttctgtgcagccttctggaagggggcttcactctaggctggtggcgtgtaaggcctcagtcttacatgccaatggagaatggcaagttctccattcatccatctgggttgaaaaggcctagcgaccagttcaagcctctccctctcatctgtagttgctaacttttcttaaacatgttgtgggaagaggagaccccagcaagtgtttcttaagtgatttcaccagtgaaacccccaggagacttttgctgggaaggctggcagtggagctcactaggaagccttcttaccaaggaaaagccttgtgttcttaggctagacagctctcctagctggagcctccttgagagccacagcagtaactgtgggcctgggacatgcccacagagagcaggtctcttcaggcaacctgggagatctagggcctactggggagggagggagccaagtctaggcaaatggagaaagtgacatttcagcaaacttgttagcacttccatggagctgtgatcagttgtccttaggagtcgaggaggagaggaagccatcacgttcacctgacctagttttctgggagaagtttctctggcagaccttgtttttagataggctcatgtctctttctccctgaacaaaggttctggctctgttaaccaagtttgggttctatgttaacctccagatgatcctgagatcaattttcataaacagggataaagaggaagaggacttggagggactggtacagcaagacctacgtttcctgtctctgccttaccccaaagaaagaactgtcagtatctttgccgctggaaggtcccagtgaagcccagagcctctgcccccagctcttggctggacacctagagatcagtcatgggtaatagtgttgaagctcaggaagcctttagacctgtcttccaacttccccactttatagccaagaaaccagacccagggcatgaagggatttgcctcaagtcacacaaatgtcacacttggggctagaatcctggtctgagttccagcccagcattcaatctcttttttcagacccattctgcatcttgcttttcttagcatagaaagtttggttgatagtgtaaacaaaatggataccactgaagatgcagagtggcacagagctcctgcctgcccacggcatcaggaggcccagcttggcaaacccttgcctgttacctgttacaggctttggtgcgggcgaagggagcagctcgaggaaaggtggtggtttcttgtacagatcaaagtccacgtggtgcctgtcccagctccacctgtctcgatccaacacaggctccagtacattagcaaacagggagttttccttccactcctcattcagctctttgatgggtggcagcttgagatcctgaaagctgctttcggtgtcgctctgaagacctgtcacttggaatcccctggctgtgagccaggcctggcgggatttcttctgggctttcttctcctcttccttcaagtccaggggctccaccatggctgagaggtaatcctgtgagtacgtgaatctctttcttggctccttggctatctcttgatacagctccttcttggcaagctctgtagaattcatggtctgggtactatagttgtagacggccttgttggcaggggctgaaattttaatcaccttcgccacggacttcggaggcttcttgctgacctggtaggcttctgtgatatttttctggatgaaactgtgctttttgtctttgttcttcataagcatggcactccgccactgcaggtacttctcctggtgggcgtggatctctaaggtgagggtggagttccgactgtggtagtcctcaagattgggggcaggctgaggtggtagggcaaacagtttctcatctgtgagttcttcttgcgaaaggggcatcccaaactcttggctcaagtcttttatcatagcagaggagggcagcaggtccctcaccgtcacgtcccagagggtggtgctgttatagcagatgtcgtggatcctggctagagcctggaagacccgcctccgctcagtgtctcgcaggaagaacaccgcctgctgcagcagcagctccgtgggctggaagaggtgcacgtggtacaggatggcctccaggtccccatagagccggctgcggaacagcagctgtgagttgtacagcaccttgtatttcctgtgttctgacctgggaatccagctttggtggttctcccacagctgcctcaagccttggtcggccaggccttccaggatgaaaaggtgtgtcttcccgtccagcaggtggaagccagtgagcacatccaggtgctgctgctcctggacccgcacacgcaccttgaaggctgacaggatctgctgcagggtcctgacagggtaggagtccaggccgagggccttagcgttgatcatggtgatgtcctgcagcaggctgtggagcagggagaccttcttaaagtcaaagacgaagatgatgcggccaaactgggagcccccaaggtcaggatcagcagctctggccccggccctcagtggcaccgcgatgtccactcgcaacttgagctgggagtcagcctctaggtagttgcccctgggcattgggccgtgctggtggccatctctggggaccccaagccccacaaccttccttctcctgctgtcctggccgcagtgtgtgggctgaacctcacagctgtggatggggacggccagattcaagtacttgtggccaaggaggaggtcagcaaaactgacctgggcgatgccataagggtaccacatcttgttctgggactcaaaggggttgttctctgtctctctgggagagatgagggcctggaagttgaggtatgaatccagagggtcctccccaaacagcacgggcttctgagaacactcctctgacttgcggtcccggtcgtgaacttccaccaccatgggggggccctccaggtattcccttaggtcactggggtgcagtgccccaaggaagatgacgttgatgtcctggaaataaacgtgggttccatggggctcccccttggtcttgtgaactggagtcttatggaactggtacttgcagtacacaggcatgcacagcctctctagttcctgaatgggtacaggctgtgatggaaggcaggaagcacacttgatctttatggtcaggggatttaaatcctgcttttgctcctcggtcatgatcggaacttctgtttttaaagtcaaaaggcaatctaaaatgttggcagacttctcactgccacgactcacgacagtttgccatccggcaaggagcggcatgacggccagctggatggagaaagcgctctgcttcctggggcctgtcagcgtggggtctgcctcttcttctgccaggggcttcttatgtctcctctggattttccttcttccctctgaatctttccctttaatttgagacctttgtctgtctaatatgtttgttaagctgctaagtgattcactctcaattaattccttgatctccatcatgcttgctcctgccaaagaaatggttggtgttcttgaaacactccattgaatcgtggaagaatcgtccattttgagggacttctcatattcctcactgttcttggaagaagtttcgggctctgcttggtgagaaccttgcaaagactttgggtgtttttctgttttttcttgttttcctggcggatgttcctggttcgactcttctctgacaatgttggtattctcaatgccctgttcagataattttctctgatttaaaaccaaatgtctcacttctgacttatgaaaagctcccacgtcgtctgtgaagccggcagtctttaatcggtaatatctgacttttcttgacatcttgtctttagtgttccagagcctcaaggtgattttgtggaaatttattttctttaataattcctttgtcacagtgatattaaaagtctgctcccacgacacccaggctttgtcaccttcgtgccacggcttcacagtcttccgccagttccacgcgcgcctctgtggctacttcg

SEQ ID NO: 14092 - RNA, 12667 nt, Homo sapiens
  source 1..12667: mol_type = other RNA
gctgggattacaggcatgagccaccgcaccgggcctgccaaggcaattttagattgagcaagtgcagagccctttgcgcaggacccctggcatctgcccagcatgcctggctgtattctcttttttttggagacatagtctcactttgtcacccaggctggctggagtgcagtggcatgatcttggctcactgcaacctccacctcctgggttcaagcaactcctgtgcctcagcctcctgagtagttgggattataggcacgcaccaccatgcccagctaatatttgtatttttagtagaaacaaacagggtttcaccatgttggccaagctggtctccaacccctgacctcaggtgatccgcccaccttggcctcccaaagtgctgggattacaggcatgagccactgtgcccagccctggctgtattcttgaagctgcccggggaaggctcacgaagggaggagcatctggttgtacctgattctggagacagcattttacctgcccctttacccactgtactccatccaaaatgaccctgcagtgccctgcagaggtctcaggccttggcctagagaacagagggctttgctcgtgctccccgctctgtctgcagtgctcttcctcttctatagccactcgaccatatctaggaatgcccagctcagtctacctctgaccctcacagtcctgttgacctgaggttctggatcagtgtccccacaaagcccagtcgtgttgccaagtgatgggtgtaggcgccagcactgtggcacttgctgagagtggcatatgattttttgcaggtcctagccctgggggtagcccagacacccccccagtgctgacaggttatgtgctgtggagggtgctgaaatggtttctcctccagtgggctggaatcacagatgggctgtttacggagcaagtgccggctccaccccatgagatctgggggttagagatgagcaggatgagtcctttgtaactgagaatgaagctgtacccctttctctccctgcagccctgaatcacttgctgggggtctggaggaggggttcacccttagggctgcttcatggtgggtgggctgactttgtggaaaaatgcccccacttcagccatgtttgtcttatcacggtgcagaaagatcacccaccatctctccttttccttcccagatgctccagaaaacctagatgagcagattaagaaagtgtcccagcagatccttgagaagcgagcctatatctgtgcccaccctctggacaggacatgctgaggcaggggacagtgtcccctgctaccgcccgcccctacccatggcccgttgctggatgactgttactcttttttcagaaggtgttgggattatcacaggttaagccttttgttccccgtctgcacctgaagggttgtcgcctggcctgggagagcctcttccaggttttgacctgcaggcagtgctctctaacaggaccatcacagcttctgaactgagccggagagagagaatggaattgctgacccctggaactggcgggtattctggtcattgaggagacaccatagtggaaactggggcttatgctgctgcctccagggtgtgaggtgggtggggacctgtgtcaggtgtggatagccatttctgctcaaccacacattctctaagaaacagcttgaaagctctgtctgggtcattcatttaaactagaagcagaggcacttaaaacatgtaccaggaaccatttaacaaagaatataaaatgtcacaatctgtgtactgttagcctttgctgtacttgtcacactgttccttagaaccagcctttaatgggtgacagcaggaccctgagaaccaccctttggtgatggcctcgggtcccctttgtcctcaccctgcaaggagggcccagaatgctaaggagcagacacacagtgcaggccacaatcccttggggttatgagcccttagtttttatccttctcaggagatgatggggaggctgtctcagctgatgatgttcccacctagggactttagtttctttacaagaactggcttctactcttgaggagaggatgaatggtatctccaggccagcaggcctttgcatttctccagcctcccttctgctggcacttgaaagattacaccaggtcccagcgtgctcactgtggtgaactttaagctttgatgtggtccttgggtggtctggagctctaaaatgcctattgtggacactcccttgagcacagagaaggcagccgactctttttcctccaagtatattcccaatttactgtgatgctggaaataggcaaggaggagactgggaacttggagagctgagctggctgagtggggctggcctgagcattctgccaggggtttggtaactagtttttaaaatggggaaagtttgtaaatattgtgaccgtgtaaataacctctcagtgaaacctgaagttctgttagtgatagcagggcagcattttgcacaaaatgaagcatgcatacctctggacagaaggctgcttagagtttctttgcacaggagaagtttggggaggggctgtcagacccaccccccttctgtgcagccttctggaagggggcttcactctaggctggtggcgtgtaaggcctcagtcttacatgccaatggagaatggcaagttctccattcatccatctgggttgaaaaggcctagcgaccagttcaagcctctccctctcatctgtagttgctaacttttcttaaacatgttgtgggaagaggagaccccagcaagtgtttcttaagtgatttcaccagtgaaacccccaggagacttttgctgggaaggctggcagtggagctcactaggaagccttcttaccaaggaaaagccttgtgttcttaggctagacagctctcctagctggagcctccttgagagccacagcagtaactgtgggcctgggacatgcccacagagagcaggtctcttcaggcaacctgggagatctagggcctactggggagggagggagccaagtctaggcaaatggagaaagtgacatttcagcaaacttgttagcacttccatggagctgtgatcagttgtccttaggagtcgaggaggagaggaagccatcacgttcacctgacctagttttctgggagaagtttctctggcagaccttgtttttagataggctcatgtctctttctccctgaacaaaggttctggctctgttaaccaagtttgggttctatgttaacctccagatgatcctgagatcaattttcataaacagggataaagaggaagaggacttggagggactggtacagcaagacctacgtttcctgtctctgccttaccccaaagaaagaactgtcagtatctttgccgctggaaggtcccagtgaagcccagagcctctgcccccagctcttggctggacacctagagatcagtcatgggtaatagtgttgaagctcaggaagcctttagacctgtcttccaacttccccactttatagccaagaaaccagacccagggcatgaagggatttgcctcaagtcacacaaatgtcacacttggggctagaatcctggtctgagttccagcccagcattcaatctcttttttcagacccattctgcatcttgcttttcttagcatagaaagtttggttgatagtgtaaacaaaatggataccactgaagatgcagagtggcacagagctcctgcctgcccacggcatcaggaggcccagcttggcaaacccttgcctgttacctgttacaggctttggtgcgggcgaagggagcagctcgaggaaaggtggtggtttcttgtacagatcaaagtccacgtggtgcctgtcccagctccacctgtctcgatccaacacaggctccagtacattagcaaacagggagttttccttccactcctcattcagctctttgatgggtggcagcttgagatcctgaaagctgctttcggtgtcgctctgaagacctgtcacttggaatcccctggctgtgagccaggcctggcgggatttcttctgggctttcttctcctcttccttcaagtccaggggctccaccatggctgagaggtaatcctgtgagtacgtgaatctctttcttggctccttggctatctcttgatacagctccttcttggcaagctctgtagaattcatggtctgggtactatagttgtagacggccttgttggcaggggctgaaattttaatcaccttcgccacggacttcggaggcttcttgctgacctggtaggcttctgtgatatttttctggatgaaactgtgctttttgtctttgttcttcataagcatggcactccgccactgcaggtacttctcctggtgggcgtggatctctaaggtgagggtggagttccgactgtggtagtcctcaagattgggggcaggctgaggtggtagggcaaacagtttctcatctgtgagttcttcttgcgaaaggggcatcccaaactcttggctcaagtcttttatcatagcagaggagggcagcaggtccctcaccgtcacgtcccagagggtggtgctgttatagcagatgtcgtggatcctggctagagcctggaagacccgcctccgctcagtgtctcgcaggaagaacaccgcctgctgcagcagcagctccgtgggctggaagaggtgcacgtggtacaggatggcctccaggtccccatagagccggctgcggaacagcagctgtgagttgtacagcaccttgtatttcctgtgttctgacctgggaatccagctttggtggttctcccacagctgcctcaagccttggtcggccaggccttccaggatgaaaaggtgtgtcttcccgtccagcaggtggaagccagtgagcacatccaggtgctgctgctcctggacccgcacacgcaccttgaaggctgacaggatctgctgcagggtcctgacagggtaggagtccaggccgagggccttagcgttgatcatggtgatgtcctgcagcaggctgtggagcagggagaccttcttaaagtcaaagacgaagatgatgcggccaaactgggagcccccaaggtcaggatcagcagctctggccccggccctcagtggcaccgcgatgtccactcgcaacttgagctgggagtcagcctctaggtagttgcccctgggcattgggccgtgctggtggccatctctggggaccccaagccccacaaccttccttctcctgctgtcctggccgcagtgtgtgggctgaacctcacagctgtggatggggacggccagattcaagtacttgtggccaaggaggaggtcagcaaaactgacctgggcgatgccataagggtaccacatcttgttctgggactcaaaggggttgttctctgtctctctgggagagatgagggcctggaagttgaggtatgaatccagagggtcctccccaaacagcacgggcttctgagaacactcctctgacttgcggtcccggtcgtgaacttccaccaccatgggggggccctccaggtattcccttaggtcactggggtgcagtgccccaaggaagatgacgttgatgtcctggaaataaacgtgggttccatggggctcccccttggtcttgtgaactggagtcttatggaactggtacttgcagtacacaggcatgcacagcctctctagttcctgaatgggtacaggctgtgatggaaggcaggaagcacacttgatctttatggtcaggggatttaaatcctgcttttgctcctcggtcatgatcggaacttctgtttttaaagtcaaaaggcaatctaaaatgttggcagacttctcactgccacgactcacgacagtttgccatccggcaaggagcggcatgacggccagctggatggagaaagcgctctgcttcctggggcctgtcagcgtggggtctgcctcttcttctgccaggggcttcttatgtctcctctggattttccttcttccctctgaatctttccctttaatttgagacctttgtctgtctaatatgtttgttaagctgctaagtgattcactctcaattaattccttgatctccatcatgcttgctcctgccaaagaaatggttggtgttcttgaaacactccattgaatcgtggaagaatcgtccattttgagggacttctcatattcctcactgttcttggaagaagtttcgggctctgcttggtgagaaccttgcaaagactttgggtgtttttctgttttttcttgttttcctggcggatgttcctggttcgactcttctctgacaatgttggtattctcaatgccctgttcagataattttctctgatttaaaaccaaatgtctcacttctgacttatgaaaagctcccacgtcgtctgtgaagccggcagtctttaatcggtaatatctgacttttcttgacatcttgtctttagtgttccagagcctcaaggtgattttgtggaaatttattttctttaataattcctttgtcacagtgatattaaaagtctgctcccacgacacccaggctttgtcaccttcgtgccacggcttcacagtctttactcctgactccaggaatactttggccaccattggaaatagcaatatgtcaacttttttaggttcttcatcgtccggcagaaggaaatactcaatgtggtaaaaacgacgcatctttgtaacagaactgtctgttttagggtgtttcttatatttttcaatcaaacttgcatattttcccttccatattcacagggaaggccagtgagatggtgaatttgcaggggaccacgtggggcacgtcggagctgaaagtgctggcaggctcagatgaggactcgatgctgctgcacgggcggtcagagtcagactcctgggccctggccttggccttcaggtgttcctccacgtcacactcgctcgtggactggtaaaagctagtgatggaggagatgggctctatgcttgcggggtcctcttcccactcccaggcatgtagcgacatgctgcagagcgcactgctggccgccggcgctcctgcgagcggatgcgctgggcggcagcggggagttggaccgcggcggcaactcccgtaccggatccacagccacctgggcgaagagactccaagactgagaggagcgtccgccggtgcagggagggccgcaggcccagccactcagctacgtttggcggttgctaggagacgcgagggcgtgcggcctgggggcggggctccgcggggcggggctttccccctcagccactgcgcgcagtttgtcaaatggctacatccaggttcagaaaccagctgccttcattccttcactcatgcattcactcattaaggagtttctactcggaacgtcagcacctactataagcctggtccttgcccgtacgatgggaggtaggggttgatggctccttcctccccctccatcagctcccacctcccattctttaataaaagcaaaggaagctgtgggctctgcaaactccagacctccccacgatccctctcattagattctctgcttctgtcgccgatgtccttaaaaaccagacctccccacgatccctctcattagattctctgcttctgtcgctgatgtccttaaaatagcatgagaattcttgttagtgatcatgagcgccaactcagagatcagaaaacaaagcttagagaggtgaagcgattcgcccgaggtcacacagcaagtagggcgcagcactgtgttgaaatccggactgcctgactccaaagcctccgctcgtctgctaaaccacccaagctgagagccctggctgcggctcctaatgtagaggacctcagcacagcaagcggctgggacagagggctggggtaggcctcatggaggaagtgagcaacgccaaatctggggggtgactaggcagaggcggtgaaagcaagagaaagcatcccaggtagaggaacagcatatgcaaaggcccatagaggtgaaagggcatggcaagtttcaggaatgggtggcgaggctgtagcagtgtgcagggcccatggtacatagccccacagggcaggttagggcacaggactatgggcaatggggagccaaggcaggtcttctgttgagggagggcaccctgctccggcagtcagtttgttcaagagaatgggagctgaggctacacacaagcttggctattaagaaaactttagctgagttgagctatgacctactttgtgtcaaagagcaaaactgtggcgcagctggggctgagacccaagtcctgagcctcccagtgcatgcctccccagaccgctctcagggcatgggacagcccctttaatactgggtgctccaatactcctcgggttcagtctgaaaaacagcctcaagtacagctgttagggaagacaccaaatggcagtgggccctgtgaggagtgggttcaaactcttagcacgagaacggcaaccaccttgcccacaccccacctgcagcagcctggagactgctgtctgtatgccaggaagtgctcaggagacacatgaagggctggaagaatacaaagctactcagatacaccagcccccaaaagggccctttaacaagggcagttcaacactaccaccactcttggacagacatcaggcctcctgctccccaggtcctacccactggcctgaggctggtttccctccaaaggttcctagatcacatcaccacctaggacagaagccaatctcttcccaagctcaatagtgagaggccagaggtcttggaccaagggccaatgtgccatcctggatgtgcactggaaacacctacatgtcaaaaatacaattctgaggcttcattaaagacctgtggaagtgactctccaggggtggagcttagaaaccagtggcagattgtattttccaaagacagccacctcaaaagatcccctcccacataatcttccggcaggcattgtgaggttcacattcctcccacccagttggggggtctagtctccttctctggaaactgggcagacctctgtgactggctcagtcaaaagagtgcagaggaaatgacactatgtgatttctgaggccaggtcatataaattccatctacctctgccctgttcttttgaggtatagtattcatgctaggaatccagctagcatgttgtgaggaagcccaagcagccatgtgaaatggccacatgaaactgttgtgactgacggttcccagccaattgcagcctcaacccccagacatatgagagtgcaagacttcaaatgatcccagccctcagtctttgagccaccctggctgacattgaggaacagaaacaagctgtctccatcatgagaaattgtagatttataagcaaattgttgctctcttaaaccactaagttttggggtgatttgttgtgcaataaataataggaacgggagccatatttttaaattaccaccaagattgtattgcacaaccagaatatggaaccactgccctgagagagatggtgtctgggtcaagacctagggcatcacaggatgaagtgagggcaaaggtgtgctacccactactcaggtatgagacagtggtgggtctacaaccctacctcagtgaagatggcttcagggctggcagatcagaagcaaaggaaggggggcttctgtttcagttatctgttactgagtaaaaaccatccccaaacttaatggtgtcaaacaaacacttgttatttctcaccactccatgcatcagctgagtagttctctgctggcctcgcctgggctcactccctatgctgtgctcagctggaggaccaacatggctggaagctgccagaagtcctcacttgcatgtctggcagttgctgctggctcttcgtgggcccgctggttcccctccatgggttcccccgcccccagtggtacaccagcttccttctatgtggtgcctcatctcctcatagcccggcctggcttcctcagatggcattctcagagcagggatcccagagggcaaagaagaagttgcaaggcctcttgggacctaggcgtggaaccagcaccatgtcactctgctacatgccattaaccaaagcaagtcatgaggctggccccacttcaaggggatgaagacatggactgtacatctggtaagcagagggacaagcatccaggggcaggaggtgttcaaggtcactgaacaatccatcccttcatccttactctgccgggtggagggttcccaagctcccacaggctatgtagaggccttcctgaagctatcccaagactctggcagctggaagcatattgggaatcagctacatacaccttcttcttgccccttccccatttttaacagctttattgaagtattttttatttaataaaatccatccatttcaagcgtagaattcaatgattttcagtaactttacctagtgctgtaatcatcatcataaattcattttagaacattttcatccccctaataagacttcatgcacatttataattaatctctgttccaactcccagtcctaggcaaccatatctactttgtttctaaaaattggccttttctagacatttcctataaattgagtcagacactgtgttctggctttgtgactggtttctttcacctaccgttatgtttccaaggtttatttatgttgaggcatgtgtcagtatttcattccttttcatgactgaataatattctattgtatggacagaccacagtttgcctatccattcatcagttaatgggcatttggcttgggcatttagacatttatgaacaacgttgctatgaacattcccacacaagtctttgtgtggatgtgttttcatctctcttgggtcgatatctaggagtggaagagttgggtcgtatggtcattttgtgattaacttcttgagaaactgccaaactatcttccacaggggctgcatcattttgtgttcccatcaacaacatgaagtttcctgtttctccaaattcttgacaagatttattgcctgttttattcactacagctattctcatgagtataatatagtatttcatcatagttttcatgtgcatttccctaacaagaatactgagattgttttatgcacatgttggctatttatacaacttctttggtgaaatgtctgtttgtatcttcacccactttttgattggattgtttgtcttcttgttactgagttgttaagagttcattgtaaattcggaatataagtcctttactgggcatatgttttacaaatattttctcctagtctcttgttcgtcatattttcttaatagtgtcttttgaagtgcaaatgttttgaactttgatgaaggtccgattcatcatttttttcttttttggatcatgcatttggtgtcgtatctaagaaatctttgactaacaacaggcctatttttaatagaagtaaagcttggtgtctgaacactaagcaaatctactaaccaagacccctaaaaacccaaaagctttatgacactgaaaataatggcccaaggacattcccagacagttctgggctctggatagaacaacacaagtttccaaaaaacaggctgataataccacaagcttataaaatatgtatactccttggcccagtaataaatcactcaagatatggcacaaactgttcacagtatggtttttgcggagaaaagctgaaaaccacctcagtgggcatctgtgggggatgacaaagcaccttatagttcatccccagggagcacagagcagcctctggagcagtgtctgcaaagaaaccacagccaagctgtttacaaagctcagttcctgtgcaaagaaagatcccaatggcgccctttccactgtgcttttcatgtcaagttgaatgagctacgatttgcacactgtaaaattcagatgtacacagtcatgcaaccactacaccatgaagatagagtatttcaatcactccaaaaagttctttcatgcccaaatacatagaaaagtctggaaataaatacatcagaaatacacagtgatcctctcttggtggcagaatggtggatgatttttgctttttagcattttcccggacctttaaaagacactttaaacaatatactatttgaaatggctcaaacaatactgaactgacttcagaaaatcatttctttgccacagccctgactctctcccacacagacacacgcccatccccccagctcatacaaaagaacgcaaggagacctctgagtttgctcactttgaaccttaaacaaaaaccttgtggatgcaaccagaattatttcagaggtgcctggtaacaccgcagggcagacagacaggcctgacagcaaaccattatcaacccttacttccctgagctgtaggggagtggaggccggcaacggctcccagcaagacatttaaaagctttcttttcaatattgactggcccaggaaagctactgttcaaaggattccttcaccagctgcagggatggggggtggggagggtgttgcactcttgcctgggctaccagctcttagggctgacatgaaataaaatcaggttctttttttttttt

SEQ ID NO: 14093 - RNA, 7272 nt, Homo sapiens
  source 1..7272: mol_type = other RNA
gctgggattacaggcatgagccaccgcaccgggcctgccaaggcaattttagattgagcaagtgcagagccctttgcgcaggacccctggcatctgcccagcatgcctggctgtattctcttttttttggagacatagtctcactttgtcacccaggctggctggagtgcagtggcatgatcttggctcactgcaacctccacctcctgggttcaagcaactcctgtgcctcagcctcctgagtagttgggattataggcacgcaccaccatgcccagctaatatttgtatttttagtagaaacaaacagggtttcaccatgttggccaagctggtctccaacccctgacctcaggtgatccgcccaccttggcctcccaaagtgctgggattacaggcatgagccactgtgcccagccctggctgtattcttgaagctgcccggggaaggctcacgaagggaggagcatctggttgtacctgattctggagacagcattttacctgcccctttacccactgtactccatccaaaatgaccctgcagtgccctgcagaggtctcaggccttggcctagagaacagagggctttgctcgtgctccccgctctgtctgcagtgctcttcctcttctatagccactcgaccatatctaggaatgcccagctcagtctacctctgaccctcacagtcctgttgacctgaggttctggatcagtgtccccacaaagcccagtcgtgttgccaagtgatgggtgtaggcgccagcactgtggcacttgctgagagtggcatatgattttttgcaggtcctagccctgggggtagcccagacacccccccagtgctgacaggttatgtgctgtggagggtgctgaaatggtttctcctccagtgggctggaatcacagatgggctgtttacggagcaagtgccggctccaccccatgagatctgggggttagagatgagcaggatgagtcctttgtaactgagaatgaagctgtacccctttctctccctgcagccctgaatcacttgctgggggtctggaggaggggttcacccttagggctgcttcatggtgggtgggctgactttgtggaaaaatgcccccacttcagccatgtttgtcttatcacggtgcagaaagatcacccaccatctctccttttccttcccagatgctccagaaaacctagatgagcagattaagaaagtgtcccagcagatccttgagaagcgagcctatatctgtgcccaccctctggacaggacatgctgaggcaggggacagtgtcccctgctaccgcccgcccctacccatggcccgttgctggatgactgttactcttttttcagaaggtgttgggattatcacaggttaagccttttgttccccgtctgcacctgaagggttgtcgcctggcctgggagagcctcttccaggttttgacctgcaggcagtgctctctaacaggaccatcacagcttctgaactgagccggagagagagaatggaattgctgacccctggaactggcgggtattctggtcattgaggagacaccatagtggaaactggggcttatgctgctgcctccagggtgtgaggtgggtggggacctgtgtcaggtgtggatagccatttctgctcaaccacacattctctaagaaacagcttgaaagctctgtctgggtcattcatttaaactagaagcagaggcacttaaaacatgtaccaggaaccatttaacaaagaatataaaatgtcacaatctgtgtactgttagcctttgctgtacttgtcacactgttccttagaaccagcctttaatgggtgacagcaggaccctgagaaccaccctttggtgatggcctcgggtcccctttgtcctcaccctgcaaggagggcccagaatgctaaggagcagacacacagtgcaggccacaatcccttggggttatgagcccttagtttttatccttctcaggagatgatggggaggctgtctcagctgatgatgttcccacctagggactttagtttctttacaagaactggcttctactcttgaggagaggatgaatggtatctccaggccagcaggcctttgcatttctccagcctcccttctgctggcacttgaaagattacaccaggtcccagcgtgctcactgtggtgaactttaagctttgatgtggtccttgggtggtctggagctctaaaatgcctattgtggacactcccttgagcacagagaaggcagccgactctttttcctccaagtatattcccaatttactgtgatgctggaaataggcaaggaggagactgggaacttggagagctgagctggctgagtggggctggcctgagcattctgccaggggtttggtaactagtttttaaaatggggaaagtttgtaaatattgtgaccgtgtaaataacctctcagtgaaacctgaagttctgttagtgatagcagggcagcattttgcacaaaatgaagcatgcatacctctggacagaaggctgcttagagtttctttgcacaggagaagtttggggaggggctgtcagacccaccccccttctgtgcagccttctggaagggggcttcactctaggctggtggcgtgtaaggcctcagtcttacatgccaatggagaatggcaagttctccattcatccatctgggttgaaaaggcctagcgaccagttcaagcctctccctctcatctgtagttgctaacttttcttaaacatgttgtgggaagaggagaccccagcaagtgtttcttaagtgatttcaccagtgaaacccccaggagacttttgctgggaaggctggcagtggagctcactaggaagccttcttaccaaggaaaagccttgtgttcttaggctagacagctctcctagctggagcctccttgagagccacagcagtaactgtgggcctgggacatgcccacagagagcaggtctcttcaggcaacctgggagatctagggcctactggggagggagggagccaagtctaggcaaatggagaaagtgacatttcagcaaacttgttagcacttccatggagctgtgatcagttgtccttaggagtcgaggaggagaggaagccatcacgttcacctgacctagttttctgggagaagtttctctggcagaccttgtttttagataggctcatgtctctttctccctgaacaaaggttctggctctgttaaccaagtttgggttctatgttaacctccagatgatcctgagatcaattttcataaacagggataaagaggaagaggacttggagggactggtacagcaagacctacgtttcctgtctctgccttaccccaaagaaagaactgtcagtatctttgccgctggaaggtcccagtgaagcccagagcctctgcccccagctcttggctggacacctagagatcagtcatgggtaatagtgttgaagctcaggaagcctttagacctgtcttccaacttccccactttatagccaagaaaccagacccagggcatgaagggatttgcctcaagtcacacaaatgtcacacttggggctagaatcctggtctgagttccagcccagcattcaatctcttttttcagacccattctgcatcttgcttttcttagcatagaaagtttggttgatagtgtaaacaaaatggataccactgaagatgcagagtggcacagagctcctgcctgcccacggcatcaggaggcccagcttggcaaacccttgcctgttacctgttacaggctttggtgcgggcgaagggagcagctcgaggaaaggtggtggtttcttgtacagatcaaagtccacgtggtgcctgtcccagctccacctgtctcgatccaacacaggctccagtacattagcaaacagggagttttccttccactcctcattcagctctttgatgggtggcagcttgagatcctgaaagctgctttcggtgtcgctctgaagacctgtcacttggaatcccctggctgtgagccaggcctggcgggatttcttctgggctttcttctcctcttccttcaagtccaggggctccaccatggctgagaggtaatcctgtgagtacgtgaatctctttcttggctccttggctatctcttgatacagctccttcttggcaagctctgtagaattcatggtctgggtactatagttgtagacggccttgttggcaggggctgaaattttaatcaccttcgccacggacttcggaggcttcttgctgacctggtaggcttctgtgatatttttctggatgaaactgtgctttttgtctttgttcttcataagcatggcactccgccactgcaggtacttctcctggtgggcgtggatctctaaggtgagggtggagttccgactgtggtagtcctcaagattgggggcaggctgaggtggtagggcaaacagtttctcatctgtgagttcttcttgcgaaaggggcatcccaaactcttggctcaagtcttttatcatagcagaggagggcagcaggtccctcaccgtcacgtcccagagggtggtgctgttatagcagatgtcgtggatcctggctagagcctggaagacccgcctccgctcagtgtctcgcaggaagaacaccgcctgctgcagcagcagctccgtgggctggaagaggtgcacgtggtacaggatggcctccaggtccccatagagccggctgcggaacagcagctgtgagttgtacagcaccttgtatttcctgtgttctgacctgggaatccagctttggtggttctcccacagctgcctcaagccttggtcggccaggccttccaggatgaaaaggtgtgtcttcccgtccagcaggtggaagccagtgagcacatccaggtgctgctgctcctggacccgcacacgcaccttgaaggctgacaggatctgctgcagggtcctgacagggtaggagtccaggccgagggccttagcgttgatcatggtgatgtcctgcagcaggctgtggagcagggagaccttcttaaagtcaaagacgaagatgatgcggccaaactgggagcccccaaggtcaggatcagcagctctggccccggccctcagtggcaccgcgatgtccactcgcaacttgagctgggagtcagcctctaggtagttgcccctgggcattgggccgtgctggtggccatctctggggaccccaagccccacaaccttccttctcctgctgtcctggccgcagtgtgtgggctgaacctcacagctgtggatggggacggccagattcaagtacttgtggccaaggaggaggtcagcaaaactgacctgggcgatgccataagggtaccacatcttgttctgggactcaaaggggttgttctctgtctctctgggagagatgagggcctggaagttgaggtatgaatccagagggtcctccccaaacagcacgggcttctgagaacactcctctgacttgcggtcccggtcgtgaacttccaccaccatgggggggccctccaggtattcccttaggtcactggggtgcagtgccccaaggaagatgacgttgatgtcctggaaataaacgtgggttccatggggctcccccttggtcttgtgaactggagtcttatggaactggtacttgcagtacacaggcatgcacagcctctctagttcctgaatgggtacaggctgtgatggaaggcaggaagcacacttgatctttatggtcaggggatttaaatcctgcttttgctcctcggtcatgatcggaacttctgtttttaaagtcaaaaggcaatctaaaatgttggcagacttctcactgccacgactcacgacagtttgccatccggcaaggagcggcatgacggccagctggatggagaaagcgctctgcttcctggggcctgtcagcgtggggtctgcctcttcttctgccaggggcttcttatgtctcctctggattttccttcttccctctgaatctttccctttaatttgagacctttgtctgtctaatatgtttgttaagctgctaagtgattcactctcaattaattccttgatctccatcatgcttgctcctgccaaagaaatggttggtgttcttgaaacactccattgaatcgtggaagaatcgtccattttgagggacttctcatattcctcactgttcttggaagaagtttcgggctctgcttggtgagaaccttgcaaagactttgggtgtttttctgttttttcttgttttcctggcggatgttcctggttcgactcttctctgacaatgttggtattctcaatgccctgttcagataattttctctgatttaaaaccaaatgtctcacttctgacttatgaaaagctcccacgtcgtctgtgaagccggcagtctttaatcggtaatatctgacttttcttgacatcttgtctttagtgttccagagcctcaaggtgattttgtggaaatttattttctttaataattcctttgtcacagtgatattaaaagtctgctcccacgacacccaggctttgtcaccttcgtgccacggcttcacagtctttactcctgactccaggaatactttggccaccattggaaatagcaatatgtcaacttttttaggttcttcatcgtccggcagaaggaaatactcaatgtggtaaaaacgacgcatctttgtaacagaactgtctgttttagggtgtttcttatatttttcaatcaaacttgcatattttcccttctgacccatattcacagggaaggccagtgagatggtgaatttgcaggggaccacgtggggcacgtcggagctgaaagtgctggcaggctcagatgaggactcgatgctgctgcacgggcggtcagagtcagactcctgggccctggccttggccttcaggtgttcctccacgtcacactcgctcgtggactggtaaaagctagtgatggaggagatgggctctatgcttgcggggtcctcttcccactcccaggcatgtagcgacatgctgcagagcgcactgctggccgccggcgctcctgcgagcggatgcgctgggcggcagcggggagttggaccgcggcggcaactcccgtaccggatccacagccacctgggcgaagagactccaagactgagaggagcgtccgccggtgcagggagggccgcaggcccagccactcagctacgtttggcggttgct

SEQ ID NO: 14094 - RNA, 7722 nt, Homo sapiens
  source 1..7722: mol_type = other RNA
gctgggattacaggcatgagccaccgcaccgggcctgccaaggcaattttagattgagcaagtgcagagccctttgcgcaggacccctggcatctgcccagcatgcctggctgtattctcttttttttggagacatagtctcactttgtcacccaggctggctggagtgcagtggcatgatcttggctcactgcaacctccacctcctgggttcaagcaactcctgtgcctcagcctcctgagtagttgggattataggcacgcaccaccatgcccagctaatatttgtatttttagtagaaacaaacagggtttcaccatgttggccaagctggtctccaacccctgacctcaggtgatccgcccaccttggcctcccaaagtgctgggattacaggcatgagccactgtgcccagccctggctgtattcttgaagctgcccggggaaggctcacgaagggaggagcatctggttgtacctgattctggagacagcattttacctgcccctttacccactgtactccatccaaaatgaccctgcagtgccctgcagaggtctcaggccttggcctagagaacagagggctttgctcgtgctccccgctctgtctgcagtgctcttcctcttctatagccactcgaccatatctaggaatgcccagctcagtctacctctgaccctcacagtcctgttgacctgaggttctggatcagtgtccccacaaagcccagtcgtgttgccaagtgatgggtgtaggcgccagcactgtggcacttgctgagagtggcatatgattttttgcaggtcctagccctgggggtagcccagacacccccccagtgctgacaggttatgtgctgtggagggtgctgaaatggtttctcctccagtgggctggaatcacagatgggctgtttacggagcaagtgccggctccaccccatgagatctgggggttagagatgagcaggatgagtcctttgtaactgagaatgaagctgtacccctttctctccctgcagccctgaatcacttgctgggggtctggaggaggggttcacccttagggctgcttcatggtgggtgggctgactttgtggaaaaatgcccccacttcagccatgtttgtcttatcacggtgcagaaagatcacccaccatctctccttttccttcccagatgctccagaaaacctagatgagcagattaagaaagtgtcccagcagatccttgagaagcgagcctatatctgtgcccaccctctggacaggacatgctgaggcaggggacagtgtcccctgctaccgcccgcccctacccatggcccgttgctggatgactgttactcttttttcagaaggtgttgggattatcacaggttaagccttttgttccccgtctgcacctgaagggttgtcgcctggcctgggagagcctcttccaggttttgacctgcaggcagtgctctctaacaggaccatcacagcttctgaactgagccggagagagagaatggaattgctgacccctggaactggcgggtattctggtcattgaggagacaccatagtggaaactggggcttatgctgctgcctccagggtgtgaggtgggtggggacctgtgtcaggtgtggatagccatttctgctcaaccacacattctctaagaaacagcttgaaagctctgtctgggtcattcatttaaactagaagcagaggcacttaaaacatgtaccaggaaccatttaacaaagaatataaaatgtcacaatctgtgtactgttagcctttgctgtacttgtcacactgttccttagaaccagcctttaatgggtgacagcaggaccctgagaaccaccctttggtgatggcctcgggtcccctttgtcctcaccctgcaaggagggcccagaatgctaaggagcagacacacagtgcaggccacaatcccttggggttatgagcccttagtttttatccttctcaggagatgatggggaggctgtctcagctgatgatgttcccacctagggactttagtttctttacaagaactggcttctactcttgaggagaggatgaatggtatctccaggccagcaggcctttgcatttctccagcctcccttctgctggcacttgaaagattacaccaggtcccagcgtgctcactgtggtgaactttaagctttgatgtggtccttgggtggtctggagctctaaaatgcctattgtggacactcccttgagcacagagaaggcagccgactctttttcctccaagtatattcccaatttactgtgatgctggaaataggcaaggaggagactgggaacttggagagctgagctggctgagtggggctggcctgagcattctgccaggggtttggtaactagtttttaaaatggggaaagtttgtaaatattgtgaccgtgtaaataacctctcagtgaaacctgaagttctgttagtgatagcagggcagcattttgcacaaaatgaagcatgcatacctctggacagaaggctgcttagagtttctttgcacaggagaagtttggggaggggctgtcagacccaccccccttctgtgcagccttctggaagggggcttcactctaggctggtggcgtgtaaggcctcagtcttacatgccaatggagaatggcaagttctccattcatccatctgggttgaaaaggcctagcgaccagttcaagcctctccctctcatctgtagttgctaacttttcttaaacatgttgtgggaagaggagaccccagcaagtgtttcttaagtgatttcaccagtgaaacccccaggagacttttgctgggaaggctggcagtggagctcactaggaagccttcttaccaaggaaaagccttgtgttcttaggctagacagctctcctagctggagcctccttgagagccacagcagtaactgtgggcctgggacatgcccacagagagcaggtctcttcaggcaacctgggagatctagggcctactggggagggagggagccaagtctaggcaaatggagaaagtgacatttcagcaaacttgttagcacttccatggagctgtgatcagttgtccttaggagtcgaggaggagaggaagccatcacgttcacctgacctagttttctgggagaagtttctctggcagaccttgtttttagataggctcatgtctctttctccctgaacaaaggttctggctctgttaaccaagtttgggttctatgttaacctccagatgatcctgagatcaattttcataaacagggataaagaggaagaggacttggagggactggtacagcaagacctacgtttcctgtctctgccttaccccaaagaaagaactgtcagtatctttgccgctggaaggtcccagtgaagcccagagcctctgcccccagctcttggctggacacctagagatcagtcatgggtaatagtgttgaagctcaggaagcctttagacctgtcttccaacttccccactttatagccaagaaaccagacccagggcatgaagggatttgcctcaagtcacacaaatgtcacacttggggctagaatcctggtctgagttccagcccagcattcaatctcttttttcagacccattctgcatcttgcttttcttagcatagaaagtttggttgatagtgtaaacaaaatggataccactgaagatgcagagtggcacagagctcctgcctgcccacggcatcaggaggcccagcttggcaaacccttgcctgttacctgttacaggctttggtgcgggcgaagggagcagctcgaggaaaggtggtggtttcttgtacagatcaaagtccacgtggtgcctgtcccagctccacctgtctcgatccaacacaggctccagtacattagcaaacagggagttttccttccactcctcattcagctctttgatgggtggcagcttgagatcctgaaagctgctttcggtgtcgctctgaagacctgtcacttggaatcccctggctgtgagccaggcctggcgggatttcttctgggctttcttctcctcttccttcaagtccaggggctccaccatggctgagaggtaatcctgtgagtacgtgaatctctttcttggctccttggctatctcttgatacagctccttcttggcaagctctgtagaattcatggtctgggtactatagttgtagacggccttgttggcaggggctgaaattttaatcaccttcgccacggacttcggaggcttcttgctgacctggtaggcttctgtgatatttttctggatgaaactgtgctttttgtctttgttcttcataagcatggcactccgccactgcaggtacttctcctggtgggcgtggatctctaaggtgagggtggagttccgactgtggtagtcctcaagattgggggcaggctgaggtggtagggcaaacagtttctcatctgtgagttcttcttgcgaaaggggcatcccaaactcttggctcaagtcttttatcatagcagaggagggcagcaggtccctcaccgtcacgtcccagagggtggtgctgttatagcagatgtcgtggatcctggctagagcctggaagacccgcctccgctcagtgtctcgcaggaagaacaccgcctgctgcagcagcagctccgtgggctggaagaggtgcacgtggtacaggatggcctccaggtccccatagagccggctgcggaacagcagctgtgagttgtacagcaccttgtatttcctgtgttctgacctgggaatccagctttggtggttctcccacagctgcctcaagccttggtcggccaggccttccaggatgaaaaggtgtgtcttcccgtccagcaggtggaagccagtgagcacatccaggtgctgctgctcctggacccgcacacgcaccttgaaggctgacaggatctgctgcagggtcctgacagggtaggagtccaggccgagggccttagcgttgatcatggtgatgtcctgcagcaggctgtggagcagggagaccttcttaaagtcaaagacgaagatgatgcggccaaactgggagcccccaaggtcaggatcagcagctctggccccggccctcagtggcaccgcgatgtccactcgcaacttgagctgggagtcagcctctaggtagttgcccctgggcattgggccgtgctggtggccatctctggggaccccaagccccacaaccttccttctcctgctgtcctggccgcagtgtgtgggctgaacctcacagctgtggatggggacggccagattcaagtacttgtggccaaggaggaggtcagcaaaactgacctgggcgatgccataagggtaccacatcttgttctgggactcaaaggggttgttctctgtctctctgggagagatgagggcctggaagttgaggtatgaatccagagggtcctccccaaacagcacgggcttctgagaacactcctctgacttgcggtcccggtcgtgaacttccaccaccatgggggggccctccaggtattcccttaggtcactggggtgcagtgccccaaggaagatgacgttgatgtcctggaaataaacgtgggttccatggggctcccccttggtcttgtgaactggagtcttatggaactggtacttgcagtacacaggcatgcacagcctctctagttcctgaatgggtacaggctgtgatggaaggcaggaagcacacttgatctttatggtcaggggatttaaatcctgcttttgctcctcggtcatgatcggaacttctgtttttaaagtcaaaaggcaatctaaaatgttggcagacttctcactgccacgactcacgacagtttgccatccggcaaggagcggcatgacggccagctggatggagaaagcgctctgcttcctggggcctgtcagcgtggggtctgcctcttcttctgccaggggcttcttatgtctcctctggattttccttcttccctctgaatctttccctttaatttgagacctttgtctgtctaatatgtttgttaagctgctaagtgattcactctcaattaattccttgatctccatcatgcttgctcctgccaaagaaatggttggtgttcttgaaacactccattgaatcgtggaagaatcgtccattttgagggacttctcatattcctcactgttcttggaagaagtttcgggctctgcttggtgagaaccttgcaaagactttgggtgtttttctgttttttcttgttttcctggcggatgttcctggttcgactcttctctgacaatgttggtattctcaatgccctgttcagataattttctctgatttaaaaccaaatgtctcacttctgacttatgaaaagctcccacgtcgtctgtgaagccggcagtctttaatcggtaatatctgacttttcttgacatcttgtctttagtgttccagagcctcaaggtgattttgtggaaatttattttctttaataattcctttgtcacagtgatattaaaagtctgctcccacgacacccaggctttgtcaccttcgtgccacggcttcacagtctttactcctgactccaggaatactttggccaccattggaaatagcaatatgtcaacttttttaggttcttcatcgtccggcagaaggaaatactcaatgtggtaaaaacgacgcatctttgtaacagaactgtctgttttagggtgtttcttatatttttcaatcaaacttgcatattttcccttctgacccatattcacagggaaggccagtgagatggtgaatttgcaggggaccacgtggggcacgtcggagctgaaagtgctggcaggctcagatgaggactcgatgctgctgcacgggcggtcagagtcagactcctgggccctggccttggccttcaggtgttcctccacgtcacactcgctcgtggactggtaaaagctagtgatggaggagatgggctctatgcttgcggggtcctcttcccactcccaggcatgtagcgacatgctgcagagcgcactgctggccgccggcgctcctgctgacatacctcctctgccaagaagctcactgccttccacagcacatccatcattcttcatcagcagttcctctacccttgagtcttggagacagtgaccttattcccttgtgtcttttcttctccaggctgtagtctggagcctgtggagtagggagatactggcacctccccagtgagatctcaactattatgacctaagctgtagtcacgcggtctcacattgaagcaagaatccccacccgggggttttcacactggttgctgctaagcaacgtgcccattctcggcttgcactgggggaccctgaatgcaggattttatgaatcagagtcatgggctcaaaaaacacgaaattccagggttagccctggctttaggcaaagcctgatccagcagctcaactgatgttactaagggtcctgtttcttttgccgtcatctttgggctctatctgcagcccccaagcatctccggacggccccctcagaggcacaacttcccgcttcgtcggtcatcatgctccgcgccctcaggcagtcagcgaaacgccggaaacgcctgcagacgcctgcagacgctccttgtgtttcattggctacccgtgcagc

SEQ ID NO: 14095 - RNA, 7300 nt, Homo sapiens
  source 1..7300: mol_type = other RNA
gctgggattacaggcatgagccaccgcaccgggcctgccaaggcaattttagattgagcaagtgcagagccctttgcgcaggacccctggcatctgcccagcatgcctggctgtattctcttttttttggagacatagtctcactttgtcacccaggctggctggagtgcagtggcatgatcttggctcactgcaacctccacctcctgggttcaagcaactcctgtgcctcagcctcctgagtagttgggattataggcacgcaccaccatgcccagctaatatttgtatttttagtagaaacaaacagggtttcaccatgttggccaagctggtctccaacccctgacctcaggtgatccgcccaccttggcctcccaaagtgctgggattacaggcatgagccactgtgcccagccctggctgtattcttgaagctgcccggggaaggctcacgaagggaggagcatctggttgtacctgattctggagacagcattttacctgcccctttacccactgtactccatccaaaatgaccctgcagtgccctgcagaggtctcaggccttggcctagagaacagagggctttgctcgtgctccccgctctgtctgcagtgctcttcctcttctatagccactcgaccatatctaggaatgcccagctcagtctacctctgaccctcacagtcctgttgacctgaggttctggatcagtgtccccacaaagcccagtcgtgttgccaagtgatgggtgtaggcgccagcactgtggcacttgctgagagtggcatatgattttttgcaggtcctagccctgggggtagcccagacacccccccagtgctgacaggttatgtgctgtggagggtgctgaaatggtttctcctccagtgggctggaatcacagatgggctgtttacggagcaagtgccggctccaccccatgagatctgggggttagagatgagcaggatgagtcctttgtaactgagaatgaagctgtacccctttctctccctgcagccctgaatcacttgctgggggtctggaggaggggttcacccttagggctgcttcatggtgggtgggctgactttgtggaaaaatgcccccacttcagccatgtttgtcttatcacggtgcagaaagatcacccaccatctctccttttccttcccagatgctccagaaaacctagatgagcagattaagaaagtgtcccagcagatccttgagaagcgagcctatatctgtgcccaccctctggacaggacatgctgaggcaggggacagtgtcccctgctaccgcccgcccctacccatggcccgttgctggatgactgttactcttttttcagaaggtgttgggattatcacaggttaagccttttgttccccgtctgcacctgaagggttgtcgcctggcctgggagagcctcttccaggttttgacctgcaggcagtgctctctaacaggaccatcacagcttctgaactgagccggagagagagaatggaattgctgacccctggaactggcgggtattctggtcattgaggagacaccatagtggaaactggggcttatgctgctgcctccagggtgtgaggtgggtggggacctgtgtcaggtgtggatagccatttctgctcaaccacacattctctaagaaacagcttgaaagctctgtctgggtcattcatttaaactagaagcagaggcacttaaaacatgtaccaggaaccatttaacaaagaatataaaatgtcacaatctgtgtactgttagcctttgctgtacttgtcacactgttccttagaaccagcctttaatgggtgacagcaggaccctgagaaccaccctttggtgatggcctcgggtcccctttgtcctcaccctgcaaggagggcccagaatgctaaggagcagacacacagtgcaggccacaatcccttggggttatgagcccttagtttttatccttctcaggagatgatggggaggctgtctcagctgatgatgttcccacctagggactttagtttctttacaagaactggcttctactcttgaggagaggatgaatggtatctccaggccagcaggcctttgcatttctccagcctcccttctgctggcacttgaaagattacaccaggtcccagcgtgctcactgtggtgaactttaagctttgatgtggtccttgggtggtctggagctctaaaatgcctattgtggacactcccttgagcacagagaaggcagccgactctttttcctccaagtatattcccaatttactgtgatgctggaaataggcaaggaggagactgggaacttggagagctgagctggctgagtggggctggcctgagcattctgccaggggtttggtaactagtttttaaaatggggaaagtttgtaaatattgtgaccgtgtaaataacctctcagtgaaacctgaagttctgttagtgatagcagggcagcattttgcacaaaatgaagcatgcatacctctggacagaaggctgcttagagtttctttgcacaggagaagtttggggaggggctgtcagacccaccccccttctgtgcagccttctggaagggggcttcactctaggctggtggcgtgtaaggcctcagtcttacatgccaatggagaatggcaagttctccattcatccatctgggttgaaaaggcctagcgaccagttcaagcctctccctctcatctgtagttgctaacttttcttaaacatgttgtgggaagaggagaccccagcaagtgtttcttaagtgatttcaccagtgaaacccccaggagacttttgctgggaaggctggcagtggagctcactaggaagccttcttaccaaggaaaagccttgtgttcttaggctagacagctctcctagctggagcctccttgagagccacagcagtaactgtgggcctgggacatgcccacagagagcaggtctcttcaggcaacctgggagatctagggcctactggggagggagggagccaagtctaggcaaatggagaaagtgacatttcagcaaacttgttagcacttccatggagctgtgatcagttgtccttaggagtcgaggaggagaggaagccatcacgttcacctgacctagttttctgggagaagtttctctggcagaccttgtttttagataggctcatgtctctttctccctgaacaaaggttctggctctgttaaccaagtttgggttctatgttaacctccagatgatcctgagatcaattttcataaacagggataaagaggaagaggacttggagggactggtacagcaagacctacgtttcctgtctctgccttaccccaaagaaagaactgtcagtatctttgccgctggaaggtcccagtgaagcccagagcctctgcccccagctcttggctggacacctagagatcagtcatgggtaatagtgttgaagctcaggaagcctttagacctgtcttccaacttccccactttatagccaagaaaccagacccagggcatgaagggatttgcctcaagtcacacaaatgtcacacttggggctagaatcctggtctgagttccagcccagcattcaatctcttttttcagacccattctgcatcttgcttttcttagcatagaaagtttggttgatagtgtaaacaaaatggataccactgaagatgcagagtggcacagagctcctgcctgcccacggcatcaggaggcccagcttggcaaacccttgcctgttacctgttacaggctttggtgcgggcgaagggagcagctcgaggaaaggtggtggtttcttgtacagatcaaagtccacgtggtgcctgtcccagctccacctgtctcgatccaacacaggctccagtacattagcaaacagggagttttccttccactcctcattcagctctttgatgggtggcagcttgagatcctgaaagctgctttcggtgtcgctctgaagacctgtcacttggaatcccctggctgtgagccaggcctggcgggatttcttctgggctttcttctcctcttccttcaagtccaggggctccaccatggctgagaggtaatcctgtgagtacgtgaatctctttcttggctccttggctatctcttgatacagctccttcttggcaagctctgtagaattcatggtctgggtactatagttgtagacggccttgttggcaggggctgaaattttaatcaccttcgccacggacttcggaggcttcttgctgacctggtaggcttctgtgatatttttctggatgaaactgtgctttttgtctttgttcttcataagcatggcactccgccactgcaggtacttctcctggtgggcgtggatctctaaggtgagggtggagttccgactgtggtagtcctcaagattgggggcaggctgaggtggtagggcaaacagtttctcatctgtgagttcttcttgcgaaaggggcatcccaaactcttggctcaagtcttttatcatagcagaggagggcagcaggtccctcaccgtcacgtcccagagggtggtgctgttatagcagatgtcgtggatcctggctagagcctggaagacccgcctccgctcagtgtctcgcaggaagaacaccgcctgctgcagcagcagctccgtgggctggaagaggtgcacgtggtacaggatggcctccaggtccccatagagccggctgcggaacagcagctgtgagttgtacagcaccttgtatttcctgtgttctgacctgggaatccagctttggtggttctcccacagctgcctcaagccttggtcggccaggccttccaggatgaaaaggtgtgtcttcccgtccagcaggtggaagccagtgagcacatccaggtgctgctgctcctggacccgcacacgcaccttgaaggctgacaggatctgctgcagggtcctgacagggtaggagtccaggccgagggccttagcgttgatcatggtgatgtcctgcagcaggctgtggagcagggagaccttcttaaagtcaaagacgaagatgatgcggccaaactgggagcccccaaggtcaggatcagcagctctggccccggccctcagtggcaccgcgatgtccactcgcaacttgagctgggagtcagcctctaggtagttgcccctgggcattgggccgtgctggtggccatctctggggaccccaagccccacaaccttccttctcctgctgtcctggccgcagtgtgtgggctgaacctcacagctgtggatggggacggccagattcaagtacttgtggccaaggaggaggtcagcaaaactgacctgggcgatgccataagggtaccacatcttgttctgggactcaaaggggttgttctctgtctctctgggagagatgagggcctggaagttgaggtatgaatccagagggtcctccccaaacagcacgggcttctgagaacactcctctgacttgcggtcccggtcgtgaacttccaccaccatgggggggccctccaggtattcccttaggtcactggggtgcagtgccccaaggaagatgacgttgatgtcctggaaataaacgtgggttccatggggctcccccttggtcttgtgaactggagtcttatggaactggtacttgcagtacacaggcatgcacagcctctctagttcctgaatgggtacaggctgtgatggaaggcaggaagcacacttgatctttatggtcaggggatttaaatcctgcttttgctcctcggtcatgatcggaacttctgtttttaaagtcaaaaggcaatctaaaatgttggcagacttctcactgccacgactcacgacagtttgccatccggcaaggagcggcatgacggccagctggatggagaaagcgctctgcttcctggggcctgtcagcgtggggtctgcctcttcttctgccaggggcttcttatgtctcctctggattttccttcttccctctgaatctttccctttaatttgagacctttgtctgtctaatatgtttgttaagctgctaagtgattcactctcaattaattccttgatctccatcatgcttgctcctgccaaagaaatggttggtgttcttgaaacactccattgaatcgtggaagaatcgtccattttgagggacttctcatattcctcactgttcttggaagaagtttcgggctctgcttggtgagaaccttgcaaagactttgggtgtttttctgttttttcttgttttcctggcggatgttcctggttcgactcttctctgacaatgttggtattctcaatgccctgttcagataattttctctgatttaaaaccaaatgtctcacttctgacttatgaaaagctcccacgtcgtctgtgaagccggcagtctttaatcggtaatatctgacttttcttgacatcttgtctttagtgttccagagcctcaaggtgattttgtggaaatttattttctttaataattcctttgtcacagtgatattaaaagtctgctcccacgacacccaggctttgtcaccttcgtgccacggcttcacagtctttactcctgactccaggaatactttggccaccattggaaatagcaatatgtcaacttttttaggttcttcatcgtccggcagaaggaaatactcaatgtggtaaaaacgacgcatctttgtaacagaactgtctgttttagggtgtttcttatatttttcaatcaaacttgcatattttcccttctgacccatattcacagggaaggccagtgagatggtgaatttgcaggggaccacgtggggcacgtcggagctgaaagtgctggcaggctcagatgaggactcgatgctgctgcacgggcggtcagagtcagactcctgggccctggccttggccttcaggtgttcctccacgtcacactcgctcgtggactggtaaaagctagtgatggaggagatgggctctatgcttgcggggtcctcttcccactcccaggcatgtagcgacatgctgcagagcgcactgctggccgccggcgctcctgctgacatacctcctctgccaagaagctcactgccttccacagcacatccatcattcttcatcagcagttcctctgagaccacaaacagggcctggcttgtgtcatcttagaaaacagggaagaagccaggcacggtggttcatgcctgtaatcccaacactttgggaggctgagacaggaggatcactt

SEQ ID NO: 14096 - RNA, 7726 nt, Homo sapiens
  source 1..7726: mol_type = other RNA
gctgggattacaggcatgagccaccgcaccgggcctgccaaggcaattttagattgagcaagtgcagagccctttgcgcaggacccctggcatctgcccagcatgcctggctgtattctcttttttttggagacatagtctcactttgtcacccaggctggctggagtgcagtggcatgatcttggctcactgcaacctccacctcctgggttcaagcaactcctgtgcctcagcctcctgagtagttgggattataggcacgcaccaccatgcccagctaatatttgtatttttagtagaaacaaacagggtttcaccatgttggccaagctggtctccaacccctgacctcaggtgatccgcccaccttggcctcccaaagtgctgggattacaggcatgagccactgtgcccagccctggctgtattcttgaagctgcccggggaaggctcacgaagggaggagcatctggttgtacctgattctggagacagcattttacctgcccctttacccactgtactccatccaaaatgaccctgcagtgccctgcagaggtctcaggccttggcctagagaacagagggctttgctcgtgctccccgctctgtctgcagtgctcttcctcttctatagccactcgaccatatctaggaatgcccagctcagtctacctctgaccctcacagtcctgttgacctgaggttctggatcagtgtccccacaaagcccagtcgtgttgccaagtgatgggtgtaggcgccagcactgtggcacttgctgagagtggcatatgattttttgcaggtcctagccctgggggtagcccagacacccccccagtgctgacaggttatgtgctgtggagggtgctgaaatggtttctcctccagtgggctggaatcacagatgggctgtttacggagcaagtgccggctccaccccatgagatctgggggttagagatgagcaggatgagtcctttgtaactgagaatgaagctgtacccctttctctccctgcagccctgaatcacttgctgggggtctggaggaggggttcacccttagggctgcttcatggtgggtgggctgactttgtggaaaaatgcccccacttcagccatgtttgtcttatcacggtgcagaaagatcacccaccatctctccttttccttcccagatgctccagaaaacctagatgagcagattaagaaagtgtcccagcagatccttgagaagcgagcctatatctgtgcccaccctctggacaggacatgctgaggcaggggacagtgtcccctgctaccgcccgcccctacccatggcccgttgctggatgactgttactcttttttcagaaggtgttgggattatcacaggttaagccttttgttccccgtctgcacctgaagggttgtcgcctggcctgggagagcctcttccaggttttgacctgcaggcagtgctctctaacaggaccatcacagcttctgaactgagccggagagagagaatggaattgctgacccctggaactggcgggtattctggtcattgaggagacaccatagtggaaactggggcttatgctgctgcctccagggtgtgaggtgggtggggacctgtgtcaggtgtggatagccatttctgctcaaccacacattctctaagaaacagcttgaaagctctgtctgggtcattcatttaaactagaagcagaggcacttaaaacatgtaccaggaaccatttaacaaagaatataaaatgtcacaatctgtgtactgttagcctttgctgtacttgtcacactgttccttagaaccagcctttaatgggtgacagcaggaccctgagaaccaccctttggtgatggcctcgggtcccctttgtcctcaccctgcaaggagggcccagaatgctaaggagcagacacacagtgcaggccacaatcccttggggttatgagcccttagtttttatccttctcaggagatgatggggaggctgtctcagctgatgatgttcccacctagggactttagtttctttacaagaactggcttctactcttgaggagaggatgaatggtatctccaggccagcaggcctttgcatttctccagcctcccttctgctggcacttgaaagattacaccaggtcccagcgtgctcactgtggtgaactttaagctttgatgtggtccttgggtggtctggagctctaaaatgcctattgtggacactcccttgagcacagagaaggcagccgactctttttcctccaagtatattcccaatttactgtgatgctggaaataggcaaggaggagactgggaacttggagagctgagctggctgagtggggctggcctgagcattctgccaggggtttggtaactagtttttaaaatggggaaagtttgtaaatattgtgaccgtgtaaataacctctcagtgaaacctgaagttctgttagtgatagcagggcagcattttgcacaaaatgaagcatgcatacctctggacagaaggctgcttagagtttctttgcacaggagaagtttggggaggggctgtcagacccaccccccttctgtgcagccttctggaagggggcttcactctaggctggtggcgtgtaaggcctcagtcttacatgccaatggagaatggcaagttctccattcatccatctgggttgaaaaggcctagcgaccagttcaagcctctccctctcatctgtagttgctaacttttcttaaacatgttgtgggaagaggagaccccagcaagtgtttcttaagtgatttcaccagtgaaacccccaggagacttttgctgggaaggctggcagtggagctcactaggaagccttcttaccaaggaaaagccttgtgttcttaggctagacagctctcctagctggagcctccttgagagccacagcagtaactgtgggcctgggacatgcccacagagagcaggtctcttcaggcaacctgggagatctagggcctactggggagggagggagccaagtctaggcaaatggagaaagtgacatttcagcaaacttgttagcacttccatggagctgtgatcagttgtccttaggagtcgaggaggagaggaagccatcacgttcacctgacctagttttctgggagaagtttctctggcagaccttgtttttagataggctcatgtctctttctccctgaacaaaggttctggctctgttaaccaagtttgggttctatgttaacctccagatgatcctgagatcaattttcataaacagggataaagaggaagaggacttggagggactggtacagcaagacctacgtttcctgtctctgccttaccccaaagaaagaactgtcagtatctttgccgctggaaggtcccagtgaagcccagagcctctgcccccagctcttggctggacacctagagatcagtcatgggtaatagtgttgaagctcaggaagcctttagacctgtcttccaacttccccactttatagccaagaaaccagacccagggcatgaagggatttgcctcaagtcacacaaatgtcacacttggggctagaatcctggtctgagttccagcccagcattcaatctcttttttcagacccattctgcatcttgcttttcttagcatagaaagtttggttgatagtgtaaacaaaatggataccactgaagatgcagagtggcacagagctcctgcctgcccacggcatcaggaggcccagcttggcaaacccttgcctgttacctgttacaggctttggtgcgggcgaagggagcagctcgaggaaaggtggtggtttcttgtacagatcaaagtccacgtggtgcctgtcccagctccacctgtctcgatccaacacaggctccagtacattagcaaacagggagttttccttccactcctcattcagctctttgatgggtggcagcttgagatcctgaaagctgctttcggtgtcgctctgaagacctgtcacttggaatcccctggctgtgagccaggcctggcgggatttcttctgggctttcttctcctcttccttcaagtccaggggctccaccatggctgagaggtaatcctgtgagtacgtgaatctctttcttggctccttggctatctcttgatacagctccttcttggcaagctctgtagaattcatggtctgggtactatagttgtagacggccttgttggcaggggctgaaattttaatcaccttcgccacggacttcggaggcttcttgctgacctggtaggcttctgtgatatttttctggatgaaactgtgctttttgtctttgttcttcataagcatggcactccgccactgcaggtacttctcctggtgggcgtggatctctaaggtgagggtggagttccgactgtggtagtcctcaagattgggggcaggctgaggtggtagggcaaacagtttctcatctgtgagttcttcttgcgaaaggggcatcccaaactcttggctcaagtcttttatcatagcagaggagggcagcaggtccctcaccgtcacgtcccagagggtggtgctgttatagcagatgtcgtggatcctggctagagcctggaagacccgcctccgctcagtgtctcgcaggaagaacaccgcctgctgcagcagcagctccgtgggctggaagaggtgcacgtggtacaggatggcctccaggtccccatagagccggctgcggaacagcagctgtgagttgtacagcaccttgtatttcctgtgttctgacctgggaatccagctttggtggttctcccacagctgcctcaagccttggtcggccaggccttccaggatgaaaaggtgtgtcttcccgtccagcaggtggaagccagtgagcacatccaggtgctgctgctcctggacccgcacacgcaccttgaaggctgacaggatctgctgcagggtcctgacagggtaggagtccaggccgagggccttagcgttgatcatggtgatgtcctgcagcaggctgtggagcagggagaccttcttaaagtcaaagacgaagatgatgcggccaaactgggagcccccaaggtcaggatcagcagctctggccccggccctcagtggcaccgcgatgtccactcgcaacttgagctgggagtcagcctctaggtagttgcccctgggcattgggccgtgctggtggccatctctggggaccccaagccccacaaccttccttctcctgctgtcctggccgcagtgtgtgggctgaacctcacagctgtggatggggacggccagattcaagtacttgtggccaaggaggaggtcagcaaaactgacctgggcgatgccataagggtaccacatcttgttctgggactcaaaggggttgttctctgtctctctgggagagatgagggcctggaagttgaggtatgaatccagagggtcctccccaaacagcacgggcttctgagaacactcctctgacttgcggtcccggtcgtgaacttccaccaccatgggggggccctccaggtattcccttaggtcactggggtgcagtgccccaaggaagatgacgttgatgtcctggaaataaacgtgggttccatggggctcccccttggtcttgtgaactggagtcttatggaactggtacttgcagtacacaggcatgcacagcctctctagttcctgaatgggtacaggctgtgatggaaggcaggaagcacacttgatctttatggtcaggggatttaaatcctgcttttgctcctcggtcatgatcggaacttctgtttttaaagtcaaaaggcaatctaaaatgttggcagacttctcactgccacgactcacgacagtttgccatccggcaaggagcggcatgacggccagctggatggagaaagcgctctgcttcctggggcctgtcagcgtggggtctgcctcttcttctgccaggggcttcttatgtctcctctggattttccttcttccctctgaatctttccctttaatttgagacctttgtctgtctaatatgtttgttaagctgctaagtgattcactctcaattaattccttgatctccatcatgcttgctcctgccaaagaaatggttggtgttcttgaaacactccattgaatcgtggaagaatcgtccattttgagggacttctcatattcctcactgttcttggaagaagtttcgggctctgcttggtgagaaccttgcaaagactttgggtgtttttctgttttttcttgttttcctggcggatgttcctggttcgactcttctctgacaatgttggtattctcaatgccctgttcagataattttctctgatttaaaaccaaatgtctcacttctgacttatgaaaagctcccacgtcgtctgtgaagccggcagtctttaatcggtaatatctgacttttcttgacatcttgtctttagtgttccagagcctcaaggtgattttgtggaaatttattttctttaataattcctttgtcacagtgatattaaaagtctgctcccacgacacccaggctttgtcaccttcgtgccacggcttcacagtctttactcctgactccaggaatactttggccaccattggaaatagcaatatgtcaacttttttaggttcttcatcgtccggcagaaggaaatactcaatgtggtaaaaacgacgcatctttgtaacagaactgtctgttttagggtgtttcttatatttttcaatcaaacttgcatattttcccttctgacccatattcacagggaaggccagtgagatggtgaatttgcaggggaccacgtggggcacgtcggagctgaaagtgctggcaggctcagatgaggactcgatgctgctgcacgggcggtcagagtcagactcctgggccctggccttggccttcaggtgttcctccacgtcacactcgctcgtggactggtaaaagctagtgatggaggagatgggctctatgcttgcggggtcctcttcccactcccaggcatgtagcgacatgctgcagagcgcactgctggccgccggcgctcctgctgacatacctcctctgccaagaagctcactgccttccacagcacatccatcattcttcatcagcagttcctgcctctacccttgagtcttggagacagtgaccttattcccttgtgtcttttcttctccaggctgtagtctggagcctgtggagtagggagatactggcacctccccagtgagatctcaactattatgacctaagctgtagtcacgcggtctcacattgaagcaagaatccccacccgggggttttcacactggttgctgctaagcaacgtgcccattctcggcttgcactgggggaccctgaatgcaggattttatgaatcagagtcatgggctcaaaaaacacgaaattccagggttagccctggctttaggcaaagcctgatccagcagctcaactgatgttactaagggtcctgtttcttttgccgtcatctttgggctctatctgcagcccccaagcatctccggacggccccctcagaggcacaacttcccgcttcgtcggtcatcatgctccgcgccctcaggcagtcagcgaaacgccggaaacgcctgcagacgcctgcagacgctccttgtgtttcattggctacccgtgcagc

SEQ ID NO: 14097 - RNA, 7693 nt, Homo sapiens
  source 1..7693: mol_type = other RNA
gctgggattacaggcatgagccaccgcaccgggcctgccaaggcaattttagattgagcaagtgcagagccctttgcgcaggacccctggcatctgcccagcatgcctggctgtattctcttttttttggagacatagtctcactttgtcacccaggctggctggagtgcagtggcatgatcttggctcactgcaacctccacctcctgggttcaagcaactcctgtgcctcagcctcctgagtagttgggattataggcacgcaccaccatgcccagctaatatttgtatttttagtagaaacaaacagggtttcaccatgttggccaagctggtctccaacccctgacctcaggtgatccgcccaccttggcctcccaaagtgctgggattacaggcatgagccactgtgcccagccctggctgtattcttgaagctgcccggggaaggctcacgaagggaggagcatctggttgtacctgattctggagacagcattttacctgcccctttacccactgtactccatccaaaatgaccctgcagtgccctgcagaggtctcaggccttggcctagagaacagagggctttgctcgtgctccccgctctgtctgcagtgctcttcctcttctatagccactcgaccatatctaggaatgcccagctcagtctacctctgaccctcacagtcctgttgacctgaggttctggatcagtgtccccacaaagcccagtcgtgttgccaagtgatgggtgtaggcgccagcactgtggcacttgctgagagtggcatatgattttttgcaggtcctagccctgggggtagcccagacacccccccagtgctgacaggttatgtgctgtggagggtgctgaaatggtttctcctccagtgggctggaatcacagatgggctgtttacggagcaagtgccggctccaccccatgagatctgggggttagagatgagcaggatgagtcctttgtaactgagaatgaagctgtacccctttctctccctgcagccctgaatcacttgctgggggtctggaggaggggttcacccttagggctgcttcatggtgggtgggctgactttgtggaaaaatgcccccacttcagccatgtttgtcttatcacggtgcagaaagatcacccaccatctctccttttccttcccagatgctccagaaaacctagatgagcagattaagaaagtgtcccagcagatccttgagaagcgagcctatatctgtgcccaccctctggacaggacatgctgaggcaggggacagtgtcccctgctaccgcccgcccctacccatggcccgttgctggatgactgttactcttttttcagaaggtgttgggattatcacaggttaagccttttgttccccgtctgcacctgaagggttgtcgcctggcctgggagagcctcttccaggttttgacctgcaggcagtgctctctaacaggaccatcacagcttctgaactgagccggagagagagaatggaattgctgacccctggaactggcgggtattctggtcattgaggagacaccatagtggaaactggggcttatgctgctgcctccagggtgtgaggtgggtggggacctgtgtcaggtgtggatagccatttctgctcaaccacacattctctaagaaacagcttgaaagctctgtctgggtcattcatttaaactagaagcagaggcacttaaaacatgtaccaggaaccatttaacaaagaatataaaatgtcacaatctgtgtactgttagcctttgctgtacttgtcacactgttccttagaaccagcctttaatgggtgacagcaggaccctgagaaccaccctttggtgatggcctcgggtcccctttgtcctcaccctgcaaggagggcccagaatgctaaggagcagacacacagtgcaggccacaatcccttggggttatgagcccttagtttttatccttctcaggagatgatggggaggctgtctcagctgatgatgttcccacctagggactttagtttctttacaagaactggcttctactcttgaggagaggatgaatggtatctccaggccagcaggcctttgcatttctccagcctcccttctgctggcacttgaaagattacaccaggtcccagcgtgctcactgtggtgaactttaagctttgatgtggtccttgggtggtctggagctctaaaatgcctattgtggacactcccttgagcacagagaaggcagccgactctttttcctccaagtatattcccaatttactgtgatgctggaaataggcaaggaggagactgggaacttggagagctgagctggctgagtggggctggcctgagcattctgccaggggtttggtaactagtttttaaaatggggaaagtttgtaaatattgtgaccgtgtaaataacctctcagtgaaacctgaagttctgttagtgatagcagggcagcattttgcacaaaatgaagcatgcatacctctggacagaaggctgcttagagtttctttgcacaggagaagtttggggaggggctgtcagacccaccccccttctgtgcagccttctggaagggggcttcactctaggctggtggcgtgtaaggcctcagtcttacatgccaatggagaatggcaagttctccattcatccatctgggttgaaaaggcctagcgaccagttcaagcctctccctctcatctgtagttgctaacttttcttaaacatgttgtgggaagaggagaccccagcaagtgtttcttaagtgatttcaccagtgaaacccccaggagacttttgctgggaaggctggcagtggagctcactaggaagccttcttaccaaggaaaagccttgtgttcttaggctagacagctctcctagctggagcctccttgagagccacagcagtaactgtgggcctgggacatgcccacagagagcaggtctcttcaggcaacctgggagatctagggcctactggggagggagggagccaagtctaggcaaatggagaaagtgacatttcagcaaacttgttagcacttccatggagctgtgatcagttgtccttaggagtcgaggaggagaggaagccatcacgttcacctgacctagttttctgggagaagtttctctggcagaccttgtttttagataggctcatgtctctttctccctgaacaaaggttctggctctgttaaccaagtttgggttctatgttaacctccagatgatcctgagatcaattttcataaacagggataaagaggaagaggacttggagggactggtacagcaagacctacgtttcctgtctctgccttaccccaaagaaagaactgtcagtatctttgccgctggaaggtcccagtgaagcccagagcctctgcccccagctcttggctggacacctagagatcagtcatgggtaatagtgttgaagctcaggaagcctttagacctgtcttccaacttccccactttatagccaagaaaccagacccagggcatgaagggatttgcctcaagtcacacaaatgtcacacttggggctagaatcctggtctgagttccagcccagcattcaatctcttttttcagacccattctgcatcttgcttttcttagcatagaaagtttggttgatagtgtaaacaaaatggataccactgaagatgcagagtggcacagagctcctgcctgcccacggcatcaggaggcccagcttggcaaacccttgcctgttacctgttacaggctttggtgcgggcgaagggagcagctcgaggaaaggtggtggtttcttgtacagatcaaagtccacgtggtgcctgtcccagctccacctgtctcgatccaacacaggctccagtacattagcaaacagggagttttccttccactcctcattcagctctttgatgggtggcagcttgagatcctgaaagctgctttcggtgtcgctctgaagacctgtcacttggaatcccctggctgtgagccaggcctggcgggatttcttctgggctttcttctcctcttccttcaagtccaggggctccaccatggctgagaggtaatcctgtgagtacgtgaatctctttcttggctccttggctatctcttgatacagctccttcttggcaagctctgtagaattcatggtctgggtactatagttgtagacggccttgttggcaggggctgaaattttaatcaccttcgccacggacttcggaggcttcttgctgacctggtaggcttctgtgatatttttctggatgaaactgtgctttttgtctttgttcttcataagcatggcactccgccactgcaggtacttctcctggtgggcgtggatctctaaggtgagggtggagttccgactgtggtagtcctcaagattgggggcaggctgaggtggtagggcaaacagtttctcatctgtgagttcttcttgcgaaaggggcatcccaaactcttggctcaagtcttttatcatagcagaggagggcagcaggtccctcaccgtcacgtcccagagggtggtgctgttatagcagatgtcgtggatcctggctagagcctggaagacccgcctccgctcagtgtctcgcaggaagaacaccgcctgctgcagcagcagctccgtgggctggaagaggtgcacgtggtacaggatggcctccaggtccccatagagccggctgcggaacagcagctgtgagttgtacagcaccttgtatttcctgtgttctgacctgggaatccagctttggtggttctcccacagctgcctcaagccttggtcggccaggccttccaggatgaaaaggtgtgtcttcccgtccagcaggtggaagccagtgagcacatccaggtgctgctgctcctggacccgcacacgcaccttgaaggctgacaggatctgctgcagggtcctgacagggtaggagtccaggccgagggccttagcgttgatcatggtgatgtcctgcagcaggctgtggagcagggagaccttcttaaagtcaaagacgaagatgatgcggccaaactgggagcccccaaggtcaggatcagcagctctggccccggccctcagtggcaccgcgatgtccactcgcaacttgagctgggagtcagcctctaggtagttgcccctgggcattgggccgtgctggtggccatctctggggaccccaagccccacaaccttccttctcctgctgtcctggccgcagtgtgtgggctgaacctcacagctgtggatggggacggccagattcaagtacttgtggccaaggaggaggtcagcaaaactgacctgggcgatgccataagggtaccacatcttgttctgggactcaaaggggttgttctctgtctctctgggagagatgagggcctggaagttgaggtatgaatccagagggtcctccccaaacagcacgggcttctgagaacactcctctgacttgcggtcccggtcgtgaacttccaccaccatgggggggccctccaggtattcccttaggtcactggggtgcagtgccccaaggaagatgacgttgatgtcctggaaataaacgtgggttccatggggctcccccttggtcttgtgaactggagtcttatggaactggtacttgcagtacacaggcatgcacagcctctctagttcctgaatgggtacaggctgtgatggaaggcaggaagcacacttgatctttatggtcaggggatttaaatcctgcttttgctcctcggtcatgatcggaacttctgtttttaaagtcaaaaggcaatctaaaatgttggcagacttctcactgccacgactcacgacagtttgccatccggcaaggagcggcatgacggccagctggatggagaaagcgctctgcttcctggggcctgtcagcgtggggtctgcctcttcttctgccaggggcttcttatgtctcctctggattttccttcttccctctgaatctttccctttaatttgagacctttgtctgtctaatatgtttgttaagctgctaagtgattcactctcaattaattccttgatctccatcatgcttgctcctgccaaagaaatggttggtgttcttgaaacactccattgaatcgtggaagaatcgtccattttgagggacttctcatattcctcactgttcttggaagaagtttcgggctctgcttggtgagaaccttgcaaagactttgggtgtttttctgttttttcttgttttcctggcggatgttcctggttcgactcttctctgacaatgttggtattctcaatgccctgttcagataattttctctgatttaaaaccaaatgtctcacttctgacttatgaaaagctcccacgtcgtctgtgaagccggcagtctttaatcggtaatatctgacttttcttgacatcttgtctttagtgttccagagcctcaaggtgattttgtggaaatttattttctttaataattcctttgtcacagtgatattaaaagtctgctcccacgacacccaggctttgtcaccttcgtgccacggcttcacagtctttactcctgactccaggaatactttggccaccattggaaatagcaatatgtcaacttttttaggttcttcatcgtccggcagaaggaaatactcaatgtggtaaaaacgacgcatctttgtaacagaactgtctgttttagggtgtttcttatatttttcaatcaaacttgcatattttcccttctgacccatattcacagggaaggccagtgagatggtgaatttgcaggggaccacgtggggcacgtcggagctgaaagtgctggcaggctcagatgaggactcgatgctgctgcacgggcggtcagagtcagactcctgggccctggccttggccttcaggtgttcctccacgtcacactcgctcgtggactggtaaaagctagtgatggaggagatgggctctatgcttgcggggtcctcttcccactcccaggcatgtagcgacatgctgcagagcgcactgctggccgccggcgctcctgctgacatacctcctctgccaagaagctcactgccttccacagcacatccatcattcttcatcagcagttccttattcccttgtgtcttttcttctccaggctgtagtctggagcctgtggagtagggagatactggcacctccccagtgagatctcaactattatgacctaagctgtagtcacgcggtctcacattgaagcaagaatccccacccgggggttttcacactggttgctgctaagcaacgtgcccattctcggcttgcactgggggaccctgaatgcaggattttatgaatcagagtcatgggctcaaaaaacacgaaattccagggttagccctggctttaggcaaagcctgatccagcagctcaactgatgttactaagggtcctgtttcttttgccgtcatctttgggctctatctgcagcccccaagcatctccggacggccccctcagaggcacaacttcccgcttcgtcggtcatcatgctccgcgccctcaggcagtcagcgaaacgccggaaacgcctgcagacgcctgcagacgctccttgtgtttcattggctacccgtgcagc

SEQ ID NO: 14098 - RNA, 12378 nt, Homo sapiens
  source 1..12378: mol_type = other RNA
gctgggattacaggcatgagccaccgcaccgggcctgccaaggcaattttagattgagcaagtgcagagccctttgcgcaggacccctggcatctgcccagcatgcctggctgtattctcttttttttggagacatagtctcactttgtcacccaggctggctggagtgcagtggcatgatcttggctcactgcaacctccacctcctgggttcaagcaactcctgtgcctcagcctcctgagtagttgggattataggcacgcaccaccatgcccagctaatatttgtatttttagtagaaacaaacagggtttcaccatgttggccaagctggtctccaacccctgacctcaggtgatccgcccaccttggcctcccaaagtgctgggattacaggcatgagccactgtgcccagccctggctgtattcttgaagctgcccggggaaggctcacgaagggaggagcatctggttgtacctgattctggagacagcattttacctgcccctttacccactgtactccatccaaaatgaccctgcagtgccctgcagaggtctcaggccttggcctagagaacagagggctttgctcgtgctccccgctctgtctgcagtgctcttcctcttctatagccactcgaccatatctaggaatgcccagctcagtctacctctgaccctcacagtcctgttgacctgaggttctggatcagtgtccccacaaagcccagtcgtgttgccaagtgatgggtgtaggcgccagcactgtggcacttgctgagagtggcatatgattttttgcaggtcctagccctgggggtagcccagacacccccccagtgctgacaggttatgtgctgtggagggtgctgaaatggtttctcctccagtgggctggaatcacagatgggctgtttacggagcaagtgccggctccaccccatgagatctgggggttagagatgagcaggatgagtcctttgtaactgagaatgaagctgtacccctttctctccctgcagccctgaatcacttgctgggggtctggaggaggggttcacccttagggctgcttcatggtgggtgggctgactttgtggaaaaatgcccccacttcagccatgtttgtcttatcacggtgcagaaagatcacccaccatctctccttttccttcccagatgctccagaaaacctagatgagcagattaagaaagtgtcccagcagatccttgagaagcgagcctatatctgtgcccaccctctggacaggacatgctgaggcaggggacagtgtcccctgctaccgcccgcccctacccatggcccgttgctggatgactgttactcttttttcagaaggtgttgggattatcacaggttaagccttttgttccccgtctgcacctgaagggttgtcgcctggcctgggagagcctcttccaggttttgacctgcaggcagtgctctctaacaggaccatcacagcttctgaactgagccggagagagagaatggaattgctgacccctggaactggcgggtattctggtcattgaggagacaccatagtggaaactggggcttatgctgctgcctccagggtgtgaggtgggtggggacctgtgtcaggtgtggatagccatttctgctcaaccacacattctctaagaaacagcttgaaagctctgtctgggtcattcatttaaactagaagcagaggcacttaaaacatgtaccaggaaccatttaacaaagaatataaaatgtcacaatctgtgtactgttagcctttgctgtacttgtcacactgttccttagaaccagcctttaatgggtgacagcaggaccctgagaaccaccctttggtgatggcctcgggtcccctttgtcctcaccctgcaaggagggcccagaatgctaaggagcagacacacagtgcaggccacaatcccttggggttatgagcccttagtttttatccttctcaggagatgatggggaggctgtctcagctgatgatgttcccacctagggactttagtttctttacaagaactggcttctactcttgaggagaggatgaatggtatctccaggccagcaggcctttgcatttctccagcctcccttctgctggcacttgaaagattacaccaggtcccagcgtgctcactgtggtgaactttaagctttgatgtggtccttgggtggtctggagctctaaaatgcctattgtggacactcccttgagcacagagaaggcagccgactctttttcctccaagtatattcccaatttactgtgatgctggaaataggcaaggaggagactgggaacttggagagctgagctggctgagtggggctggcctgagcattctgccaggggtttggtaactagtttttaaaatggggaaagtttgtaaatattgtgaccgtgtaaataacctctcagtgaaacctgaagttctgttagtgatagcagggcagcattttgcacaaaatgaagcatgcatacctctggacagaaggctgcttagagtttctttgcacaggagaagtttggggaggggctgtcagacccaccccccttctgtgcagccttctggaagggggcttcactctaggctggtggcgtgtaaggcctcagtcttacatgccaatggagaatggcaagttctccattcatccatctgggttgaaaaggcctagcgaccagttcaagcctctccctctcatctgtagttgctaacttttcttaaacatgttgtgggaagaggagaccccagcaagtgtttcttaagtgatttcaccagtgaaacccccaggagacttttgctgggaaggctggcagtggagctcactaggaagccttcttaccaaggaaaagccttgtgttcttaggctagacagctctcctagctggagcctccttgagagccacagcagtaactgtgggcctgggacatgcccacagagagcaggtctcttcaggcaacctgggagatctagggcctactggggagggagggagccaagtctaggcaaatggagaaagtgacatttcagcaaacttgttagcacttccatggagctgtgatcagttgtccttaggagtcgaggaggagaggaagccatcacgttcacctgacctagttttctgggagaagtttctctggcagaccttgtttttagataggctcatgtctctttctccctgaacaaaggttctggctctgttaaccaagtttgggttctatgttaacctccagatgatcctgagatcaattttcataaacagggataaagaggaagaggacttggagggactggtacagcaagacctacgtttcctgtctctgccttaccccaaagaaagaactgtcagtatctttgccgctggaaggtcccagtgaagcccagagcctctgcccccagctcttggctggacacctagagatcagtcatgggtaatagtgttgaagctcaggaagcctttagacctgtcttccaacttccccactttatagccaagaaaccagacccagggcatgaagggatttgcctcaagtcacacaaatgtcacacttggggctagaatcctggtctgagttccagcccagcattcaatctcttttttcagacccattctgcatcttgcttttcttagcatagaaagtttggttgatagtgtaaacaaaatggataccactgaagatgcagagtggcacagagctcctgcctgcccacggcatcaggaggcccagcttggcaaacccttgcctgttacctgttacaggctttggtgcgggcgaagggagcagctcgaggaaaggtggtggtttcttgtacagatcaaagtccacgtggtgcctgtcccagctccacctgtctcgatccaacacaggctccagtacattagcaaacagggagttttccttccactcctcattcagctctttgatgggtggcagcttgagatcctgaaagctgctttcggtgtcgctctgaagacctgtcacttggaatcccctggctgtgagccaggcctggcgggatttcttctgggctttcttctcctcttccttcaagtccaggggctccaccatggctgagaggtaatcctgtgagtacgtgaatctctttcttggctccttggctatctcttgatacagctccttcttggcaagctctgtagaattcatggtctgggtactatagttgtagacggccttgttggcaggggctgaaattttaatcaccttcgccacggacttcggaggcttcttgctgacctggtaggcttctgtgatatttttctggatgaaactgtgctttttgtctttgttcttcataagcatggcactccgccactgcaggtacttctcctggtgggcgtggatctctaaggtgagggtggagttccgactgtggtagtcctcaagattgggggcaggctgaggtggtagggcaaacagtttctcatctgtgagttcttcttgcgaaaggggcatcccaaactcttggctcaagtcttttatcatagcagaggagggcagcaggtccctcaccgtcacgtcccagagggtggtgctgttatagcagatgtcgtggatcctggctagagcctggaagacccgcctccgctcagtgtctcgcaggaagaacaccgcctgctgcagcagcagctccgtgggctggaagaggtgcacgtggtacaggatggcctccaggtccccatagagccggctgcggaacagcagctgtgagttgtacagcaccttgtatttcctgtgttctgacctgggaatccagctttggtggttctcccacagctgcctcaagccttggtcggccaggccttccaggatgaaaaggtgtgtcttcccgtccagcaggtggaagccagtgagcacatccaggtgctgctgctcctggacccgcacacgcaccttgaaggctgacaggatctgctgcagggtcctgacagggtaggagtccaggccgagggccttagcgttgatcatggtgatgtcctgcagcaggctgtggagcagggagaccttcttaaagtcaaagacgaagatgatgcggccaaactgggagcccccaaggtcaggatcagcagctctggccccggccctcagtggcaccgcgatgtccactcgcaacttgagctgggagtcagcctctaggtagttgcccctgggcattgggccgtgctggtggccatctctggggaccccaagccccacaaccttccttctcctgctgtcctggccgcagtgtgtgggctgaacctcacagctgtggatggggacggccagattcaagtacttgtggccaaggaggaggtcagcaaaactgacctgggcgatgccataagggtaccacatcttgttctgggactcaaaggggttgttctctgtctctctgggagagatgagggcctggaagttgaggtatgaatccagagggtcctccccaaacagcacgggcttctgagaacactcctctgacttgcggtcccggtcgtgaacttccaccaccatgggggggccctccaggtattcccttaggtcactggggtgcagtgccccaaggaagatgacgttgatgtcctggaaataaacgtgggttccatggggctcccccttggtcttgtgaactggagtcttatggaactggtacttgcagtacacaggcatgcacagcctctctagttcctgaatgggtacaggctgtgatggaaggcaggaagcacacttgatctttatggtcaggggatttaaatcctgcttttgctcctcggtcatgatcggaacttctgtttttaaagtcaaaaggcaatctaaaatgttggcagacttctcactgccacgactcacgacagtttgccatccggcaaggagcggcatgacggccagctggatggagaaagcgctctgcttcctggggcctgtcagcgtggggtctgcctcttcttctgccaggggcttcttatgtctcctctggattttccttcttccctctgaatctttccctttaatttgagacctttgtctgtctaatatgtttgttaagctgctaagtgattcactctcaattaattccttgatctccatcatgcttgctcctgccaaagaaatggttggtgttcttgaaacactccattgaatcgtggaagaatcgtccattttgagggacttctcatattcctcactgttcttggaagaagtttcgggctctgcttggtgagaaccttgcaaagactttgggtgtttttctgttttttcttgttttcctggcggatgttcctggttcgactcttctctgacaatgttggtattctcaatgccctgttcagataattttctctgatttaaaaccaaatgtctcacttctgacttatgaaaagctcccacgtcgtctgtgaagccggcagtctttaatcggtaatatctgacttttcttgacatcttgtctttagtgttccagagcctcaaggtgattttgtggaaatttattttctttaataattcctttgtcacagtgatattaaaagtctgctcccacgacacccaggctttgtcaccttcgtgccacggcttcacagtctttactcctgactccaggaatactttggccaccattggaaatagcaatatgtcaacttttttaggttcttcatcgtccggcagaaggaaatactcaatgtggtaaaaacgacgcatctttgtaacagaactgtctgttttagggtgtttcttatatttttcaatcaaacttgcatattttcccttctgacctgcgagcggatgcgctgggcggcagcggggagttggaccgcggcggcaactcccgtaccggatccacagccacctgggcgaagagactccaagactgagaggagcgtccgccggtgcagggagggccgcaggcccagccactcagctacgtttggcggttgctaggagacgcgagggcgtgcggcctgggggcggggctccgcggggcggggctttccccctcagccactgcgcgcagtttgtcaaatggctacatccaggttcagaaaccagctgccttcattccttcactcatgcattcactcattaaggagtttctactcggaacgtcagcacctactataagcctggtccttgcccgtacgatgggaggtaggggttgatggctccttcctccccctccatcagctcccacctcccattctttaataaaagcaaaggaagctgtgggctctgcaaactccagacctccccacgatccctctcattagattctctgcttctgtcgccgatgtccttaaaaaccagacctccccacgatccctctcattagattctctgcttctgtcgctgatgtccttaaaatagcatgagaattcttgttagtgatcatgagcgccaactcagagatcagaaaacaaagcttagagaggtgaagcgattcgcccgaggtcacacagcaagtagggcgcagcactgtgttgaaatccggactgcctgactccaaagcctccgctcgtctgctaaaccacccaagctgagagccctggctgcggctcctaatgtagaggacctcagcacagcaagcggctgggacagagggctggggtaggcctcatggaggaagtgagcaacgccaaatctggggggtgactaggcagaggcggtgaaagcaagagaaagcatcccaggtagaggaacagcatatgcaaaggcccatagaggtgaaagggcatggcaagtttcaggaatgggtggcgaggctgtagcagtgtgcagggcccatggtacatagccccacagggcaggttagggcacaggactatgggcaatggggagccaaggcaggtcttctgttgagggagggcaccctgctccggcagtcagtttgttcaagagaatgggagctgaggctacacacaagcttggctattaagaaaactttagctgagttgagctatgacctactttgtgtcaaagagcaaaactgtggcgcagctggggctgagacccaagtcctgagcctcccagtgcatgcctccccagaccgctctcagggcatgggacagcccctttaatactgggtgctccaatactcctcgggttcagtctgaaaaacagcctcaagtacagctgttagggaagacaccaaatggcagtgggccctgtgaggagtgggttcaaactcttagcacgagaacggcaaccaccttgcccacaccccacctgcagcagcctggagactgctgtctgtatgccaggaagtgctcaggagacacatgaagggctggaagaatacaaagctactcagatacaccagcccccaaaagggccctttaacaagggcagttcaacactaccaccactcttggacagacatcaggcctcctgctccccaggtcctacccactggcctgaggctggtttccctccaaaggttcctagatcacatcaccacctaggacagaagccaatctcttcccaagctcaatagtgagaggccagaggtcttggaccaagggccaatgtgccatcctggatgtgcactggaaacacctacatgtcaaaaatacaattctgaggcttcattaaagacctgtggaagtgactctccaggggtggagcttagaaaccagtggcagattgtattttccaaagacagccacctcaaaagatcccctcccacataatcttccggcaggcattgtgaggttcacattcctcccacccagttggggggtctagtctccttctctggaaactgggcagacctctgtgactggctcagtcaaaagagtgcagaggaaatgacactatgtgatttctgaggccaggtcatataaattccatctacctctgccctgttcttttgaggtatagtattcatgctaggaatccagctagcatgttgtgaggaagcccaagcagccatgtgaaatggccacatgaaactgttgtgactgacggttcccagccaattgcagcctcaacccccagacatatgagagtgcaagacttcaaatgatcccagccctcagtctttgagccaccctggctgacattgaggaacagaaacaagctgtctccatcatgagaaattgtagatttataagcaaattgttgctctcttaaaccactaagttttggggtgatttgttgtgcaataaataataggaacgggagccatatttttaaattaccaccaagattgtattgcacaaccagaatatggaaccactgccctgagagagatggtgtctgggtcaagacctagggcatcacaggatgaagtgagggcaaaggtgtgctacccactactcaggtatgagacagtggtgggtctacaaccctacctcagtgaagatggcttcagggctggcagatcagaagcaaaggaaggggggcttctgtttcagttatctgttactgagtaaaaaccatccccaaacttaatggtgtcaaacaaacacttgttatttctcaccactccatgcatcagctgagtagttctctgctggcctcgcctgggctcactccctatgctgtgctcagctggaggaccaacatggctggaagctgccagaagtcctcacttgcatgtctggcagttgctgctggctcttcgtgggcccgctggttcccctccatgggttcccccgcccccagtggtacaccagcttccttctatgtggtgcctcatctcctcatagcccggcctggcttcctcagatggcattctcagagcagggatcccagagggcaaagaagaagttgcaaggcctcttgggacctaggcgtggaaccagcaccatgtcactctgctacatgccattaaccaaagcaagtcatgaggctggccccacttcaaggggatgaagacatggactgtacatctggtaagcagagggacaagcatccaggggcaggaggtgttcaaggtcactgaacaatccatcccttcatccttactctgccgggtggagggttcccaagctcccacaggctatgtagaggccttcctgaagctatcccaagactctggcagctggaagcatattgggaatcagctacatacaccttcttcttgccccttccccatttttaacagctttattgaagtattttttatttaataaaatccatccatttcaagcgtagaattcaatgattttcagtaactttacctagtgctgtaatcatcatcataaattcattttagaacattttcatccccctaataagacttcatgcacatttataattaatctctgttccaactcccagtcctaggcaaccatatctactttgtttctaaaaattggccttttctagacatttcctataaattgagtcagacactgtgttctggctttgtgactggtttctttcacctaccgttatgtttccaaggtttatttatgttgaggcatgtgtcagtatttcattccttttcatgactgaataatattctattgtatggacagaccacagtttgcctatccattcatcagttaatgggcatttggcttgggcatttagacatttatgaacaacgttgctatgaacattcccacacaagtctttgtgtggatgtgttttcatctctcttgggtcgatatctaggagtggaagagttgggtcgtatggtcattttgtgattaacttcttgagaaactgccaaactatcttccacaggggctgcatcattttgtgttcccatcaacaacatgaagtttcctgtttctccaaattcttgacaagatttattgcctgttttattcactacagctattctcatgagtataatatagtatttcatcatagttttcatgtgcatttccctaacaagaatactgagattgttttatgcacatgttggctatttatacaacttctttggtgaaatgtctgtttgtatcttcacccactttttgattggattgtttgtcttcttgttactgagttgttaagagttcattgtaaattcggaatataagtcctttactgggcatatgttttacaaatattttctcctagtctcttgttcgtcatattttcttaatagtgtcttttgaagtgcaaatgttttgaactttgatgaaggtccgattcatcatttttttcttttttggatcatgcatttggtgtcgtatctaagaaatctttgactaacaacaggcctatttttaatagaagtaaagcttggtgtctgaacactaagcaaatctactaaccaagacccctaaaaacccaaaagctttatgacactgaaaataatggcccaaggacattcccagacagttctgggctctggatagaacaacacaagtttccaaaaaacaggctgataataccacaagcttataaaatatgtatactccttggcccagtaataaatcactcaagatatggcacaaactgttcacagtatggtttttgcggagaaaagctgaaaaccacctcagtgggcatctgtgggggatgacaaagcaccttatagttcatccccagggagcacagagcagcctctggagcagtgtctgcaaagaaaccacagccaagctgtttacaaagctcagttcctgtgcaaagaaagatcccaatggcgccctttccactgtgcttttcatgtcaagttgaatgagctacgatttgcacactgtaaaattcagatgtacacagtcatgcaaccactacaccatgaagatagagtatttcaatcactccaaaaagttctttcatgcccaaatacatagaaaagtctggaaataaatacatcagaaatacacagtgatcctctcttggtggcagaatggtggatgatttttgctttttagcattttcccggacctttaaaagacactttaaacaatatactatttgaaatggctcaaacaatactgaactgacttcagaaaatcatttctttgccacagccctgactctctcccacacagacacacgcccatccccccagctcatacaaaagaacgcaaggagacctctgagtttgctcactttgaaccttaaacaaaaaccttgtggatgcaaccagaattatttcagaggtgcctggtaacaccgcagggcagacagacaggcctgacagcaaaccattatcaacccttacttccctgagctgtaggggagtggaggccggcaacggctcccagcaagacatttaaaagctttcttttcaatattgactggcccaggaaagctactgttcaaaggattccttcaccagctgcagggatggggggtggggagggtgttgcactcttgcctgggctaccagctcttagggctgacatgaaataaaatcaggttctttttttttttt

SEQ ID NO: 14099 - RNA, 6883 nt, Homo sapiens
  source 1..6883: mol_type = other RNA
gctgggattacaggcatgagccaccgcaccgggcctgccaaggcaattttagattgagcaagtgcagagccctttgcgcaggacccctggcatctgcccagcatgcctggctgtattctcttttttttggagacatagtctcactttgtcacccaggctggctggagtgcagtggcatgatcttggctcactgcaacctccacctcctgggttcaagcaactcctgtgcctcagcctcctgagtagttgggattataggcacgcaccaccatgcccagctaatatttgtatttttagtagaaacaaacagggtttcaccatgttggccaagctggtctccaacccctgacctcaggtgatccgcccaccttggcctcccaaagtgctgggattacaggcatgagccactgtgcccagccctggctgtattcttgaagctgcccggggaaggctcacgaagggaggagcatctggttgtacctgattctggagacagcattttacctgcccctttacccactgtactccatccaaaatgaccctgcagtgccctgcagaggtctcaggccttggcctagagaacagagggctttgctcgtgctccccgctctgtctgcagtgctcttcctcttctatagccactcgaccatatctaggaatgcccagctcagtctacctctgaccctcacagtcctgttgacctgaggttctggatcagtgtccccacaaagcccagtcgtgttgccaagtgatgggtgtaggcgccagcactgtggcacttgctgagagtggcatatgattttttgcaggtcctagccctgggggtagcccagacacccccccagtgctgacaggttatgtgctgtggagggtgctgaaatggtttctcctccagtgggctggaatcacagatgggctgtttacggagcaagtgccggctccaccccatgagatctgggggttagagatgagcaggatgagtcctttgtaactgagaatgaagctgtacccctttctctccctgcagccctgaatcacttgctgggggtctggaggaggggttcacccttagggctgcttcatggtgggtgggctgactttgtggaaaaatgcccccacttcagccatgtttgtcttatcacggtgcagaaagatcacccaccatctctccttttccttcccagatgctccagaaaacctagatgagcagattaagaaagtgtcccagcagatccttgagaagcgagcctatatctgtgcccaccctctggacaggacatgctgaggcaggggacagtgtcccctgctaccgcccgcccctacccatggcccgttgctggatgactgttactcttttttcagaaggtgttgggattatcacaggttaagccttttgttccccgtctgcacctgaagggttgtcgcctggcctgggagagcctcttccaggttttgacctgcaggcagtgctctctaacaggaccatcacagcttctgaactgagccggagagagagaatggaattgctgacccctggaactggcgggtattctggtcattgaggagacaccatagtggaaactggggcttatgctgctgcctccagggtgtgaggtgggtggggacctgtgtcaggtgtggatagccatttctgctcaaccacacattctctaagaaacagcttgaaagctctgtctgggtcattcatttaaactagaagcagaggcacttaaaacatgtaccaggaaccatttaacaaagaatataaaatgtcacaatctgtgtactgttagcctttgctgtacttgtcacactgttccttagaaccagcctttaatgggtgacagcaggaccctgagaaccaccctttggtgatggcctcgggtcccctttgtcctcaccctgcaaggagggcccagaatgctaaggagcagacacacagtgcaggccacaatcccttggggttatgagcccttagtttttatccttctcaggagatgatggggaggctgtctcagctgatgatgttcccacctagggactttagtttctttacaagaactggcttctactcttgaggagaggatgaatggtatctccaggccagcaggcctttgcatttctccagcctcccttctgctggcacttgaaagattacaccaggtcccagcgtgctcactgtggtgaactttaagctttgatgtggtccttgggtggtctggagctctaaaatgcctattgtggacactcccttgagcacagagaaggcagccgactctttttcctccaagtatattcccaatttactgtgatgctggaaataggcaaggaggagactgggaacttggagagctgagctggctgagtggggctggcctgagcattctgccaggggtttggtaactagtttttaaaatggggaaagtttgtaaatattgtgaccgtgtaaataacctctcagtgaaacctgaagttctgttagtgatagcagggcagcattttgcacaaaatgaagcatgcatacctctggacagaaggctgcttagagtttctttgcacaggagaagtttggggaggggctgtcagacccaccccccttctgtgcagccttctggaagggggcttcactctaggctggtggcgtgtaaggcctcagtcttacatgccaatggagaatggcaagttctccattcatccatctgggttgaaaaggcctagcgaccagttcaagcctctccctctcatctgtagttgctaacttttcttaaacatgttgtgggaagaggagaccccagcaagtgtttcttaagtgatttcaccagtgaaacccccaggagacttttgctgggaaggctggcagtggagctcactaggaagccttcttaccaaggaaaagccttgtgttcttaggctagacagctctcctagctggagcctccttgagagccacagcagtaactgtgggcctgggacatgcccacagagagcaggtctcttcaggcaacctgggagatctagggcctactggggagggagggagccaagtctaggcaaatggagaaagtgacatttcagcaaacttgttagcacttccatggagctgtgatcagttgtccttaggagtcgaggaggagaggaagccatcacgttcacctgacctagttttctgggagaagtttctctggcagaccttgtttttagataggctcatgtctctttctccctgaacaaaggttctggctctgttaaccaagtttgggttctatgttaacctccagatgatcctgagatcaattttcataaacagggataaagaggaagaggacttggagggactggtacagcaagacctacgtttcctgtctctgccttaccccaaagaaagaactgtcagtatctttgccgctggaaggtcccagtgaagcccagagcctctgcccccagctcttggctggacacctagagatcagtcatgggtaatagtgttgaagctcaggaagcctttagacctgtcttccaacttccccactttatagccaagaaaccagacccagggcatgaagggatttgcctcaagtcacacaaatgtcacacttggggctagaatcctggtctgagttccagcccagcattcaatctcttttttcagacccattctgcatcttgcttttcttagcatagaaagtttggttgatagtgtaaacaaaatggataccactgaagatgcagagtggcacagagctcctgcctgcccacggcatcaggaggcccagcttggcaaacccttgcctgttacctgttacaggctttggtgcgggcgaagggagcagctcgaggaaaggtggtggtttcttgtacagatcaaagtccacgtggtgcctgtcccagctccacctgtctcgatccaacacaggctccagtacattagcaaacagggagttttccttccactcctcattcagctctttgatgggtggcagcttgagatcctgaaagctgctttcggtgtcgctctgaagacctgtcacttggaatcccctggctgtgagccaggcctggcgggatttcttctgggctttcttctcctcttccttcaagtccaggggctccaccatggctgagaggtaatcctgtgagtacgtgaatctctttcttggctccttggctatctcttgatacagctccttcttggcaagctctgtagaattcatggtctgggtactatagttgtagacggccttgttggcaggggctgaaattttaatcaccttcgccacggacttcggaggcttcttgctgacctggtaggcttctgtgatatttttctggatgaaactgtgctttttgtctttgttcttcataagcatggcactccgccactgcaggtacttctcctggtgggcgtggatctctaaggtgagggtggagttccgactgtggtagtcctcaagattgggggcaggctgaggtggtagggcaaacagtttctcatctgtgagttcttcttgcgaaaggggcatcccaaactcttggctcaagtcttttatcatagcagaggagggcagcaggtccctcaccgtcacgtcccagagggtggtgctgttatagcagatgtcgtggatcctggctagagcctggaagacccgcctccgctcagtgtctcgcaggaagaacaccgcctgctgcagcagcagctccgtgggctggaagaggtgcacgtggtacaggatggcctccaggtccccatagagccggctgcggaacagcagctgtgagttgtacagcaccttgtatttcctgtgttctgacctgggaatccagctttggtggttctcccacagctgcctcaagccttggtcggccaggccttccaggatgaaaaggtgtgtcttcccgtccagcaggtggaagccagtgagcacatccaggtgctgctgctcctggacccgcacacgcaccttgaaggctgacaggatctgctgcagggtcctgacagggtaggagtccaggccgagggccttagcgttgatcatggtgatgtcctgcagcaggctgtggagcagggagaccttcttaaagtcaaagacgaagatgatgcggccaaactgggagcccccaaggtcaggatcagcagctctggccccggccctcagtggcaccgcgatgtccactcgcaacttgagctgggagtcagcctctaggtagttgcccctgggcattgggccgtgctggtggccatctctggggaccccaagccccacaaccttccttctcctgctgtcctggccgcagtgtgtgggctgaacctcacagctgtggatggggacggccagattcaagtacttgtggccaaggaggaggtcagcaaaactgacctgggcgatgccataagggtaccacatcttgttctgggactcaaaggggttgttctctgtctctctgggagagatgagggcctggaagttgaggtatgaatccagagggtcctccccaaacagcacgggcttctgagaacactcctctgacttgcggtcccggtcgtgaacttccaccaccatgggggggccctccaggtattcccttaggtcactggggtgcagtgccccaaggaagatgacgttgatgtcctggaaataaacgtgggttccatggggctcccccttggtcttgtgaactggagtcttatggaactggtacttgcagtacacaggcatgcacagcctctctagttcctgaatgggtacaggctgtgatggaaggcaggaagcacacttgatctttatggtcaggggatttaaatcctgcttttgctcctcggtcatgatcggaacttctgtttttaaagtcaaaaggcaatctaaaatgttggcagacttctcactgccacgactcacgacagtttgccatccggcaaggagcggcatgacggccagctggatggagaaagcgctctgcttcctggggcctgtcagcgtggggtctgcctcttcttctgccaggggcttcttatgtctcctctggattttccttcttccctctgaatctttccctttaatttgagacctttgtctgtctaatatgtttgttaagctgctaagtgattcactctcaattaattccttgatctccatcatgcttgctcctgccaaagaaatggttggtgttcttgaaacactccattgaatcgtggaagaatcgtccattttgagggacttctcatattcctcactgttcttggaagaagtttcgggctctgcttggtgagaaccttgcaaagactttgggtgtttttctgttttttcttgttttcctggcggatgttcctggttcgactcttctctgacaatgttggtattctcaatgccctgttcagataattttctctgatttaaaaccaaatgtctcacttctgacttatgaaaagctcccacgtcgtctgtgaagccggcagtctttaatcggtaatatctgacttttcttgacatcttgtctttagtgttccagagcctcaaggtgattttgtggaaatttattttctttaataattcctttgtcacagtgatattaaaagtctgctcccacgacacccaggctttgtcaccttcgtgccacggcttcacagtctttactcctgactccaggaatactttggccaccattggaaatagcaatatgtcaacttttttaggttcttcatcgtccggcagaaggaaatactcaatgtggtaaaaacgacgcatctttgtaacagaactgtctgttttagggtgtttcttatatttttcaatcaaacttgcatattttcccttctgacctgctgacatacctcctctgccaagaagctcactgccttccacagcacatccatcattcttcatcagca

SEQ ID NO: 14100 - RNA, 6944 nt, Homo sapiens
  source 1..6944: mol_type = other RNA
gctgggattacaggcatgagccaccgcaccgggcctgccaaggcaattttagattgagcaagtgcagagccctttgcgcaggacccctggcatctgcccagcatgcctggctgtattctcttttttttggagacatagtctcactttgtcacccaggctggctggagtgcagtggcatgatcttggctcactgcaacctccacctcctgggttcaagcaactcctgtgcctcagcctcctgagtagttgggattataggcacgcaccaccatgcccagctaatatttgtatttttagtagaaacaaacagggtttcaccatgttggccaagctggtctccaacccctgacctcaggtgatccgcccaccttggcctcccaaagtgctgggattacaggcatgagccactgtgcccagccctggctgtattcttgaagctgcccggggaaggctcacgaagggaggagcatctggttgtacctgattctggagacagcattttacctgcccctttacccactgtactccatccaaaatgaccctgcagtgccctgcagaggtctcaggccttggcctagagaacagagggctttgctcgtgctccccgctctgtctgcagtgctcttcctcttctatagccactcgaccatatctaggaatgcccagctcagtctacctctgaccctcacagtcctgttgacctgaggttctggatcagtgtccccacaaagcccagtcgtgttgccaagtgatgggtgtaggcgccagcactgtggcacttgctgagagtggcatatgattttttgcaggtcctagccctgggggtagcccagacacccccccagtgctgacaggttatgtgctgtggagggtgctgaaatggtttctcctccagtgggctggaatcacagatgggctgtttacggagcaagtgccggctccaccccatgagatctgggggttagagatgagcaggatgagtcctttgtaactgagaatgaagctgtacccctttctctccctgcagccctgaatcacttgctgggggtctggaggaggggttcacccttagggctgcttcatggtgggtgggctgactttgtggaaaaatgcccccacttcagccatgtttgtcttatcacggtgcagaaagatcacccaccatctctccttttccttcccagatgctccagaaaacctagatgagcagattaagaaagtgtcccagcagatccttgagaagcgagcctatatctgtgcccaccctctggacaggacatgctgaggcaggggacagtgtcccctgctaccgcccgcccctacccatggcccgttgctggatgactgttactcttttttcagaaggtgttgggattatcacaggttaagccttttgttccccgtctgcacctgaagggttgtcgcctggcctgggagagcctcttccaggttttgacctgcaggcagtgctctctaacaggaccatcacagcttctgaactgagccggagagagagaatggaattgctgacccctggaactggcgggtattctggtcattgaggagacaccatagtggaaactggggcttatgctgctgcctccagggtgtgaggtgggtggggacctgtgtcaggtgtggatagccatttctgctcaaccacacattctctaagaaacagcttgaaagctctgtctgggtcattcatttaaactagaagcagaggcacttaaaacatgtaccaggaaccatttaacaaagaatataaaatgtcacaatctgtgtactgttagcctttgctgtacttgtcacactgttccttagaaccagcctttaatgggtgacagcaggaccctgagaaccaccctttggtgatggcctcgggtcccctttgtcctcaccctgcaaggagggcccagaatgctaaggagcagacacacagtgcaggccacaatcccttggggttatgagcccttagtttttatccttctcaggagatgatggggaggctgtctcagctgatgatgttcccacctagggactttagtttctttacaagaactggcttctactcttgaggagaggatgaatggtatctccaggccagcaggcctttgcatttctccagcctcccttctgctggcacttgaaagattacaccaggtcccagcgtgctcactgtggtgaactttaagctttgatgtggtccttgggtggtctggagctctaaaatgcctattgtggacactcccttgagcacagagaaggcagccgactctttttcctccaagtatattcccaatttactgtgatgctggaaataggcaaggaggagactgggaacttggagagctgagctggctgagtggggctggcctgagcattctgccaggggtttggtaactagtttttaaaatggggaaagtttgtaaatattgtgaccgtgtaaataacctctcagtgaaacctgaagttctgttagtgatagcagggcagcattttgcacaaaatgaagcatgcatacctctggacagaaggctgcttagagtttctttgcacaggagaagtttggggaggggctgtcagacccaccccccttctgtgcagccttctggaagggggcttcactctaggctggtggcgtgtaaggcctcagtcttacatgccaatggagaatggcaagttctccattcatccatctgggttgaaaaggcctagcgaccagttcaagcctctccctctcatctgtagttgctaacttttcttaaacatgttgtgggaagaggagaccccagcaagtgtttcttaagtgatttcaccagtgaaacccccaggagacttttgctgggaaggctggcagtggagctcactaggaagccttcttaccaaggaaaagccttgtgttcttaggctagacagctctcctagctggagcctccttgagagccacagcagtaactgtgggcctgggacatgcccacagagagcaggtctcttcaggcaacctgggagatctagggcctactggggagggagggagccaagtctaggcaaatggagaaagtgacatttcagcaaacttgttagcacttccatggagctgtgatcagttgtccttaggagtcgaggaggagaggaagccatcacgttcacctgacctagttttctgggagaagtttctctggcagaccttgtttttagataggctcatgtctctttctccctgaacaaaggttctggctctgttaaccaagtttgggttctatgttaacctccagatgatcctgagatcaattttcataaacagggataaagaggaagaggacttggagggactggtacagcaagacctacgtttcctgtctctgccttaccccaaagaaagaactgtcagtatctttgccgctggaaggtcccagtgaagcccagagcctctgcccccagctcttggctggacacctagagatcagtcatgggtaatagtgttgaagctcaggaagcctttagacctgtcttccaacttccccactttatagccaagaaaccagacccagggcatgaagggatttgcctcaagtcacacaaatgtcacacttggggctagaatcctggtctgagttccagcccagcattcaatctcttttttcagacccattctgcatcttgcttttcttagcatagaaagtttggttgatagtgtaaacaaaatggataccactgaagatgcagagtggcacagagctcctgcctgcccacggcatcaggaggcccagcttggcaaacccttgcctgttacctgttacaggctttggtgcgggcgaagggagcagctcgaggaaaggtggtggtttcttgtacagatcaaagtccacgtggtgcctgtcccagctccacctgtctcgatccaacacaggctccagtacattagcaaacagggagttttccttccactcctcattcagctctttgatgggtggcagcttgagatcctgaaagctgctttcggtgtcgctctgaagacctgtcacttggaatcccctggctgtgagccaggcctggcgggatttcttctgggctttcttctcctcttccttcaagtccaggggctccaccatggctgagaggtaatcctgtgagtacgtgaatctctttcttggctccttggctatctcttgatacagctccttcttggcaagctctgtagaattcatggtctgggtactatagttgtagacggccttgttggcaggggctgaaattttaatcaccttcgccacggacttcggaggcttcttgctgacctggtaggcttctgtgatatttttctggatgaaactgtgctttttgtctttgttcttcataagcatggcactccgccactgcaggtacttctcctggtgggcgtggatctctaaggtgagggtggagttccgactgtggtagtcctcaagattgggggcaggctgaggtggtagggcaaacagtttctcatctgtgagttcttcttgcgaaaggggcatcccaaactcttggctcaagtcttttatcatagcagaggagggcagcaggtccctcaccgtcacgtcccagagggtggtgctgttatagcagatgtcgtggatcctggctagagcctggaagacccgcctccgctcagtgtctcgcaggaagaacaccgcctgctgcagcagcagctccgtgggctggaagaggtgcacgtggtacaggatggcctccaggtccccatagagccggctgcggaacagcagctgtgagttgtacagcaccttgtatttcctgtgttctgacctgggaatccagctttggtggttctcccacagctgcctcaagccttggtcggccaggccttccaggatgaaaaggtgtgtcttcccgtccagcaggtggaagccagtgagcacatccaggtgctgctgctcctggacccgcacacgcaccttgaaggctgacaggatctgctgcagggtcctgacagggtaggagtccaggccgagggccttagcgttgatcatggtgatgtcctgcagcaggctgtggagcagggagaccttcttaaagtcaaagacgaagatgatgcggccaaactgggagcccccaaggtcaggatcagcagctctggccccggccctcagtggcaccgcgatgtccactcgcaacttgagctgggagtcagcctctaggtagttgcccctgggcattgggccgtgctggtggccatctctggggaccccaagccccacaaccttccttctcctgctgtcctggccgcagtgtgtgggctgaacctcacagctgtggatggggacggccagattcaagtacttgtggccaaggaggaggtcagcaaaactgacctgggcgatgccataagggtaccacatcttgttctgggactcaaaggggttgttctctgtctctctgggagagatgagggcctggaagttgaggtatgaatccagagggtcctccccaaacagcacgggcttctgagaacactcctctgacttgcggtcccggtcgtgaacttccaccaccatgggggggccctccaggtattcccttaggtcactggggtgcagtgccccaaggaagatgacgttgatgtcctggaaataaacgtgggttccatggggctcccccttggtcttgtgaactggagtcttatggaactggtacttgcagtacacaggcatgcacagcctctctagttcctgaatgggtacaggctgtgatggaaggcaggaagcacacttgatctttatggtcaggggatttaaatcctgcttttgctcctcggtcatgatcggaacttctgtttttaaagtcaaaaggcaatctaaaatgttggcagacttctcactgccacgactcacgacagtttgccatccggcaaggagcggcatgacggccagctggatggagaaagcgctctgcttcctggggcctgtcagcgtggggtctgcctcttcttctgccaggggcttcttatgtctcctctggattttccttcttccctctgaatctttccctttaatttgagacctttgtctgtctaatatgtttgttaagctgctaagtgattcactctcaattaattccttgatctccatcatgcttgctcctgccaaagaaatggttggtgttcttgaaacactccattgaatcgtggaagaatcgtccattttgagggacttctcatattcctcactgttcttggaagaagtttcgggctctgcttggtgagaaccttgcaaagactttgggtgtttttctgttttttcttgttttcctggcggatgttcctggttcgactcttctctgacaatgttggtattctcaatgccctgttcagataattttctctgatttaaaaccaaatgtctcacttctgacttatgaaaagctcccacgtcgtctgtgaagccggcagtctttaatcggtaatatctgacttttcttgacatcttgtctttagtgttccagagcctcaaggtgattttgtggaaatttattttctttaataattcctttgtcacagtgatattaaaagtctgctcccacgacacccaggctttgtcaccttcgtgccacggcttcacagtctttactcctgactccaggaatactttggccaccattggaaatagcaatatgtcaacttttttaggttcttcatcgtccggcagaaggaaatactcaatgtggtaaaaacgacgcatctttgtaacagaactgtctgttttagggtgtttcttatatttttcaatcaaacttgcatattttcccttctgacgtcagcagcgtgcaccagcaaaatagcagaagcaggaggagagccggctggaatacacctaccccatattcacagggaaggccagtgagatggtgaatttgcaggggaccacgtggggcacgtcggagct

SEQ ID NO: 14101 - RNA, 2215 nt, Homo sapiens
  source 1..2215: mol_type = other RNA
gctgggattacaggcatgagccaccgcaccgggtcagtgtttccatttttgccactgcagtgctgcttgtcttcaggggctgaggtgccctccccccgccccaaggaagcctctggcgccagtgcctgtctctgaaggagaatgtgggccttgcctccctgcaccagtcatacgcatggccccagtggcttggctcagagtctggcactgcaggccgactgcctccaggcacagctgcaggaagtgttccaggagcgggaatggagtggggtctgcaggagtcccaggacctggggggtgcagggctcgcacgctgaggacacccacctgcgcctgtctctggctggatgcagccacccgttgtctccctgcagccccagctgtaggtgctggggggccctggggggagctaggtgggtgggagtgcagcttcaggggtgggagagtgggcggggccctggaggcgctcctgggggctggcagggactgagctgcagacagcatcagaggggtgggggtcccacagggtcgggcaggggtagtcctgggtgtaaccggaagcagttgctgaccctgtgggggtgggggtgagggtgggagtcctcagggccctcccagagcagtccgagctgtggggtgggaggagagagggtgggaggacccagggctgggaggggagtggtcaggaggacctgggggctgggggagctcctagggcctgggcaccgcacacagggcctgggccctcggcctcatggtaaaagcccgggcgggcgtggtgtccagggaggccggactgacgccaggcgggggcagcaggcggtacctctgcaggaggccggcaaacagcaggaagagctcggtcctggccaggcgctccccaacacagacgcggcggcctgcagagaaaggcaggaaggcctcccgcttcacaaagtgcccattcgcgtccaggaaatggccggggttgaactggcctggggtctgccactgtgtctcatccaggagcaccgaggtcagcaggggaatcacgggcgtgcccttggggagcaggaagccgcccagctgtgtgtcggccgcggtgcagcggggcacgtgcggcaggagcgtgatgaaccgctgcacctcgtggagcacggcgcttgtgtagggcagagcctgctggtcctccagccggggagtccgcccagggcccagcacgcggtctagctcctcctgcacccggccctgcacgtccgggtgccggcccatcagaagtgcggcccactgcagcgtggccgaggtcgtctccgtcccggccatgaccatgtccagggtgcaggccaccgcgttggcctcagcaaacaggccctcggggtcatccccctgtccctgctggatcagggcgtccacatagctgcacacggggtcccccgggcacacgtggggcctccgcgcctccaggagggtcctcagaatggcacggacctcctcgatcttgcgcaggacgggccggtgcagctggagcagggccccgagccatgggtagacgttgaacagctgcaggccaggggaccccaagaggaccatgacctcatcgatgagacccagcagggacacaaacacggggtcccggtagtcaaatcggcggccgaagaggagcgcgaaggtgatattggagggagcccagcccagtagggccagcgggaagggccggcctctgtagccatccagctgcccagagaggcatttcagctcctgcagaatcttgtcagccaccggctcccggcccacgcccaggctgtgcagggcacgcaccgtgaactggcgggcagccctccagcgcgccccagatgagaagaagatgcctccacctcgctggatgagctggaagatggcgatgggaggccggtcggccagctcctgcccggggcccgccagcgcctctttgaccgcctcgaaccccgtcagcaccaccgtcttctggcgccccaggtgcacggtgaacaccggcccgtagcgttctgagagctccatcagggaccggtcctgttgcgacagacgcagcaagtgcaggttcccgacgagcggcagcgggcgaggccccgggggccaccgggcagctggggaggggtcttgggcgcaggcgcagagcagcccccagagccccaggaggcccaggaacagcaagagcagcagggccatgaggacgtggctggtgaggctccactcccct

SEQ ID NO: 14102 - RNA, 1822 nt, Homo sapiens
  source 1..1822: mol_type = other RNA
gctgggattacaggcatgagccaccgcaccgggtcagtgtttccatttttgccactgcagtgctgcttgtcttcaggggctgaggtgccctccccccgccccaaggaagcctctggcgccagtgcctgtctctgaaggagaatgtgggccttgcctccctgcaccagtcatacgcatggccccagtggcttggctcagagtctggcactgcaggccgactgcctccaggcacagctgcaggaagtgttccaggagcgggaatggagtggggtctgcaggagtcccaggacctggggggtgcagggctcgcacgctgaggacacccacctgcgcctgtctctggctggatgcagccacccgttgtctccctgcagccccagctgtaggtgctggggggccctggggggagctctgcaggaggccggcaaacagcaggaagagctcggtcctggccaggcgctccccaacacagacgcggcggcctgcagagaaaggcaggaaggcctcccgcttcacaaagtgcccattcgcgtccaggaaatggccggggttgaactggcctggggtctgccactgtgtctcatccaggagcaccgaggtcagcaggggaatcacgggcgtgcccttggggagcaggaagccgcccagctgtgtgtcggccgcggtgcagcggggcacgtgcggcaggagcgtgatgaaccgctgcacctcgtggagcacggcgcttgtgtagggcagagcctgctggtcctccagccggggagtccgcccagggcccagcacgcggtctagctcctcctgcacccggccctgcacgtccgggtgccggcccatcagaagtgcggcccactgcagcgtggccgaggtcgtctccgtcccggccatgaccatgtccagggtgcaggccaccgcgttggcctcagcaaacaggccctcggggtcatccccctgtccctgctggatcagggcgtccacatagctgcacacggggtcccccgggcacacgtggggcctccgcgcctccaggagggtcctcagaatggcacggacctcctcgatcttgcgcaggacgggccggtgcagctggagcagggccccgagccatgggtagacgttgaacagctgcaggccaggggaccccaagaggaccatgacctcatcgatgagacccagcagggacacaaacacggggtcccggtagtcaaatcggcggccgaagaggagcgcgaaggtgatattggagggagcccagcccagtagggccagcgggaagggccggcctctgtagccatccagctgcccagagaggcatttcagctcctgcagaatcttgtcagccaccggctcccggcccacgcccaggctgtgcagggcacgcaccgtgaactggcgggcagccctccagcgcgccccagatgagaagaagatgcctccacctcgctggatgagctggaagatggcgatgggaggccggtcggccagctcctgcccggggcccgccagcgcctctttgaccgcctcgaaccccgtcagcaccaccgtcttctggcgccccaggtgcacggtgaacaccggcccgtagcgttctgagagctccatcagggaccggtcctgttgcgacagacgcagcaagtgcaggttcccgacgagcggcagcgggcgaggccccgggggccaccgggcagctggggaggggtcttgggcgcaggcgcagagcagcccccagagccccaggaggcccaggaacagcaagagcagcagggccatgaggacgtggctggtgaggctccactcccctcctgggccccgtcccccccgcacc

SEQ ID NO: 14103 - RNA, 4958 nt, Homo sapiens
  source 1..4958: mol_type = other RNA
gctgggattacaggcatgagccaccgcacctagccggcaaacttttttaaatggttggcgggggtgggggaaatcaaatgagtaatgttttgtgacacatcaaaattataatgatgtgctgcataacttttggtcaacaatggccaaatatacgatgatgatcccgtaagattacaatggagctgaaaaattcctattgcctggggacacagccatggtaacatcatagtgaaattactttatgtagcctaagtatatagtgtttataaaagtctacagtagtgcacagtaatatcatggccttcacattcactaaccacttactgactcacccagagccagcttccagtcctgccaacttgttcatggtaaatgtcctaaataggtgtaccattttatatcttatatatatctatatatatatttttactgtaccttttctatgtttagatatgtttagatacacaaatacttagcactgtgttacaaccgcctacagtaatcagtacagtaatatgccatacaggtttgtaggttaggagcaataggctatcccatataggataccatagggtataccatctaggtttgtgtaactacatcatgattttcacacaatgatgaaattgccaagtgacatgtctcagaacatatccctgtcattaagtgacatatgactatatatgaaacttaacaaatcaggccttgttgaaacacagtcatgttgatttgtttacatattgtatatggctccttacacactatcaacggcagagttgtgtactatagttgcaatacagaccatagccaacaaagtctaaaatgttctagcacttcacagaaaaggttttttgactcctactctactgtttcagtgtcactgacccattttacctggaccaaagactactcaagtctattttcctccaactgacacaagtttctgcctcagtgtatggaggttttcctcagtaataggaaactggaaaaattagtcaacatttattgagtgcctaaatgactacctatttagtatacctgctgatttacttggcaggcttttctcactatactgcaagctccttgaaggcagagataatttacttgagtggaacctggcacaacgtaagtgctttagaaattgaataagccaagtaaaatgttttaaggcaaccctatcccaaaatattcctgaagatattaatttaatcattactaatctctgtgattagcaagggaagtagtcagtctggcacaccaaattttattaataatacttattttaatctgttccctttagtatgtctttatacagttcccctcgtgtatatacactgatataactacaatttaaaagccactaattaatctgttttttattttgtaagtaacaagatatagacatttgaatgccaatgtcttattctggagagacactggagctgaagttcaacaatgatcacacttattacctggcaataaaaacacaaccatctttccagtcaggtcaaaatatcctactttttgcctttctaccaattcccaaacattcacagtttttcaaggaccactaataaaatacaggaagcttttaaagacagtaagagaacacctagtgtaagttaggtgaattaaagatggcaaaggagattacatcctcaacactgacagcttccaagacttagaaaagagattgttccttgcttctaaaattgttctattttcctctgtaggaaaatgaaagttttttcttacaaatattaaataatcaaagtacttacgcaaaattaatctgctcctcaatgagatgagcactccatttaaatgatctttacagatccctgaagttgctgtcctgtcactgtatttaagtgatggatattcaattgaattattctgcataaataattctgttcaacccagaagtatagtagtatgatgggtcagatacagtcaactgttcaataaaaatgcagatgtctgaaattattaaaatgtacttaaaagtaacaaactgtatcacacacttaggcttagaagtgttctttcaagttttttcttttaaaaaagaaaccagtctttgaagatttttgttgaatatagctattttccaagcttcatcttctttttctttggtccattaaggtccatgtttgaagtatcagtaggaatgcttattcctggtatctgtggttctaccagggacattcggatcttctgatgttgaagattagatgagtctaacatgattttcactttaactttatcaaatacatggaacactgtatcttctattttaagtgagggtatctcatcatcataaataagctgtgggtttggtttgtccttttcttcaaaaaagactgtcccttctaaaccatactttggaattaataccacaatggcattctttcttacaaataaaatataggcttcttcacttactattcctttgcttttgaagaataactgggtatgaaaagccactgatgcacgttgggcatattgagccattttgtgccggaaatttagatttttacatatatctgcaagcttgtgtttgtctgtcaactctggataagtacagtcagccccaatagccacagccaaaagccgatgaacaatgacatctgcgtatcttctaatgggtgaagtaaaatgtgtgtatattggagacgctaagccatagtgatgaaaatcattatccattccagaacagaagtacacagcttgcatcatacagcgagtggctaatattctcaacagagtgtttagatatggaaaagtaggagattcggcctgatccaaagactcagccaaagacttggctgtatcagtcttaatttccaaattccttgacctggctgccttaacaagaatttcataatttgatggaggtggagcaggatgttttcgaagcagagcatgttcagaaaattcctcatgaattttttttgcaacagaaatattggcaagtaacataaattcttcaaccatggaatttgtttccctaagttccttggtctgcagatctataggatcgtgagtttcactgtccatgtggaatcgaacttcaggagaggatagagtcaaagcccctttttcaatccttcttttcttcagaattttggctagtttattcagtccacggagactagtggtaatatcatcattcatgtttgctgaatcaattctcaactgagcttcagcatacgtcagagatgcctttgaattaataacacttttggtaaacttcgtttttaagatttcagcattgtgattcatttcccaaatacatgaaaatgccagcctgtccacgtcacattttaaggaacacaagttagagctaagcaactctggaaccatgtcaatcctcttttcacaaagatacacagttgttcctcttctggctgattcttgatccaaggcatttcctggcctaataaaatggctcacatcagcaatatgaacaccaacctccaaatttccattttcgagttctcgacaatgtagagcatcgtctatatcagtacatcctggtgggtctacactacaaatacacagatgcctcaggtcttctcggtttttcatgtccttttcagtaatgctccagggcatctttggcagaaaactaagaacagcctgtgaaaaaggctgatggggaacatcgtgttcaagtaacaaaacttctgtttcagtctctttctctccaacatcacctaaatttctcacaaagtgtccatttggatatctggaatttctgggccaaccatcaatagcaacaataattctccgtccttctaatgtggaagcctgtctggtttctatgcgaattcgagggattctcttatcagcaggtgtaaagagatgtcttcttgactccttaatgtcagacttggaaagcatgccacaatatggtctccaattcctttttattattcctacaactctacctgtaggcttcaacattttctcgcttacagcagtcttaagcattcgttctgtctcttcttctttctccacatcttcttcattttgaccttcatcatgtaaaaccacagaagatggtgctacccactgactcttggggagaagctccacagccacaatatcttcgtgaacagctctgtttaaatgtttaagtccctgtaagattatctctttattttcttcattgtcgccatgaatccatactgtagcttccaagtaattttccctgctagctctaaatgttccttgaaggtatgtaccagattttatgccttgctgtagcttacttaagggaagatgctctgaaaatattatttttccactttctatttcattcccttcttcagacaaacaagcaagacgatctatgagttcggggttagcagttaggctctttacatattcttcacaagtgaaagctggtattccttcttctatggctttctctttgtttctcctgtcatttgttatgaagataacttgcagctggttgtctgctgacatttttttcaaatgttcattgtaccattttgctgctactcgaatcgctctatcattcctgtcattagcattttctccctgttcttgttctacataggtttctaagctgcctgggagtcgcaggctggaggccacagaagcccaggtccccggcctccaggcacttacaatctggtgcagtaacacattagtgtcgggcagcaagtagtgcggttgcgggcagacgctgctcgccgggtcctggggctgcggctccagggccggcccctcgtgcgcccctccacacgctgcgcacccgggcgcaccgcagccgatgtcgtctcgcaggtagtgctcgcgcacgatcttcatcacgccgcccgcccgggtcttttttaagaacgtcttggacttgagcatcttgcctcgccgcgcagaatcctaaccccagcagcgctcttccagcaaaaggcgtcaatctagaatac

SEQ ID NO: 14104 - RNA, 5116 nt, Homo sapiens
  source 1..5116: mol_type = other RNA
gctgggattacaggcatgagccaccgcacctagccggcaaacttttttaaatggttggcgggggtgggggaaatcaaatgagtaatgttttgtgacacatcaaaattataatgatgtgctgcataacttttggtcaacaatggccaaatatacgatgatgatcccgtaagattacaatggagctgaaaaattcctattgcctggggacacagccatggtaacatcatagtgaaattactttatgtagcctaagtatatagtgtttataaaagtctacagtagtgcacagtaatatcatggccttcacattcactaaccacttactgactcacccagagccagcttccagtcctgccaacttgttcatggtaaatgtcctaaataggtgtaccattttatatcttatatatatctatatatatatttttactgtaccttttctatgtttagatatgtttagatacacaaatacttagcactgtgttacaaccgcctacagtaatcagtacagtaatatgccatacaggtttgtaggttaggagcaataggctatcccatataggataccatagggtataccatctaggtttgtgtaactacatcatgattttcacacaatgatgaaattgccaagtgacatgtctcagaacatatccctgtcattaagtgacatatgactatatatgaaacttaacaaatcaggccttgttgaaacacagtcatgttgatttgtttacatattgtatatggctccttacacactatcaacggcagagttgtgtactatagttgcaatacagaccatagccaacaaagtctaaaatgttctagcacttcacagaaaaggttttttgactcctactctactgtttcagtgtcactgacccattttacctggaccaaagactactcaagtctattttcctccaactgacacaagtttctgcctcagtgtatggaggttttcctcagtaataggaaactggaaaaattagtcaacatttattgagtgcctaaatgactacctatttagtatacctgctgatttacttggcaggcttttctcactatactgcaagctccttgaaggcagagataatttacttgagtggaacctggcacaacgtaagtgctttagaaattgaataagccaagtaaaatgttttaaggcaaccctatcccaaaatattcctgaagatattaatttaatcattactaatctctgtgattagcaagggaagtagtcagtctggcacaccaaattttattaataatacttattttaatctgttccctttagtatgtctttatacagttcccctcgtgtatatacactgatataactacaatttaaaagccactaattaatctgttttttattttgtaagtaacaagatatagacatttgaatgccaatgtcttattctggagagacactggagctgaagttcaacaatgatcacacttattacctggcaataaaaacacaaccatctttccagtcaggtcaaaatatcctactttttgcctttctaccaattcccaaacattcacagtttttcaaggaccactaataaaatacaggaagcttttaaagacagtaagagaacacctagtgtaagttaggtgaattaaagatggcaaaggagattacatcctcaacactgacagcttccaagacttagaaaagagattgttccttgcttctaaaattgttctattttcctctgtaggaaaatgaaagttttttcttacaaatattaaataatcaaagtacttacgcaaaattaatctgctcctcaatgagatgagcactccatttaaatgatctttacagatccctgaagttgctgtcctgtcactgtatttaagtgatggatattcaattgaattattctgcataaataattctgttcaacccagaagtatagtagtatgatgggtcagatacagtcaactgttcaataaaaatgcagatgtctgaaattattaaaatgtacttaaaagtaacaaactgtatcacacacttaggcttagaagtgttctttcaagttttttcttttaaaaaagaaaccagtctttgaagatttttgttgaatatagctattttccaagcttcatcttctttttctttggtccattaaggtccatgtttgaagtatcagtaggaatgcttattcctggtatctgtggttctaccagggacattcggatcttctgatgttgaagattagatgagtctaacatgattttcactttaactttatcaaatacatggaacactgtatcttctattttaagtgagggtatctcatcatcataaataagctgtgggtttggtttgtccttttcttcaaaaaagactgtcccttctaaaccatactttggaattaataccacaatggcattctttcttacaaataaaatataggcttcttcacttactattcctttgcttttgaagaataactgggtatgaaaagccactgatgcacgttgggcatattgagccattttgtgccggaaatttagatttttacatatatctgcaagcttgtgtttgtctgtcaactctggataagtacagtcagccccaatagccacagccaaaagccgatgaacaatgacatctgcgtatcttctaatgggtgaagtaaaatgtgtgtatattggagacgctaagccatagtgatgaaaatcattatccattccagaacagaagtacacagcttgcatcatacagcgagtggctaatattctcaacagagtgtttagatatggaaaagtaggagattcggcctgatccaaagactcagccaaagacttggctgtatcagtcttaatttccaaattccttgacctggctgccttaacaagaatttcataatttgatggaggtggagcaggatgttttcgaagcagagcatgttcagaaaattcctcatgaattttttttgcaacagaaatattggcaagtaacataaattcttcaaccatggaatttgtttccctaagttccttggtctgcagatctataggatcgtgagtttcactgtccatgtggaatcgaacttcaggagaggatagagtcaaagcccctttttcaatccttcttttcttcagaattttggctagtttattcagtccacggagactagtggtaatatcatcattcatgtttgctgaatcaattctcaactgagcttcagcatacgtcagagatgcctttgaattaataacacttttggtaaacttcgtttttaagatttcagcattgtgattcatttcccaaatacatgaaaatgccagcctgtccacgtcacattttaaggaacacaagttagagctaagcaactctggaaccatgtcaatcctcttttcacaaagatacacagttgttcctcttctggctgattcttgatccaaggcatttcctggcctaataaaatggctcacatcagcaatatgaacaccaacctccaaatttccattttcgagttctcgacaatgtagagcatcgtctatatcagtacatcctggtgggtctacactacaaatacacagatgcctcaggtcttctcggtttttcatgtccttttcagtaatgctccagggcatctttggcagaaaactaagaacagcctgtgaaaaaggctgatggggaacatcgtgttcaagtaacaaaacttctgtttcagtctctttctctccaacatcacctaaatttctcacaaagtgtccatttggatatctggaatttctgggccaaccatcaatagcaacaataattctccgtccttctaatgtggaagcctgtctggtttctatgcgaattcgagggattctcttatcagcaggtgtaaagagatgtcttcttgactccttaatgtcagacttggaaagcatgccacaatatggtctccaattcctttttattattcctacaactctacctgtaggcttcaacattttctcgcttacagcagtcttaagcattcgttctgtctcttcttctttctccacatcttcttcattttgaccttcatcatgtaaaaccacagaagatggtgctacccactgactcttggggagaagctccacagccacaatatcttcgtgaacagctctgtttaaatgtttaagtccctgtaagattatctctttattttcttcattgtcgccatgaatccatactgtagcttccaagtaattttccctgctagctctaaatgttccttgaaggtatgtaccagattttatgccttgctgtagcttacttaagggaagatgctctgaaaatattatttttccactttctatttcattcccttcttcagacaaacaagcaagacgatctatgagttcggggttagcagttaggctctttacatattcttcacaagtgaaagctggtattccttcttctatggctttctctttgtttctcctgtcatttgttatgaagataacttgcagctggttgtctgctgacatttttttcaaatgttcattgtaccattttgctgctactcgaatcgctctatcattcctgtcattagcattttctccctgttcttgttctacataggtttctctatggtgctcattagtgaaagtatagaaatgcttctcttggttattagtcacatctcggatgcgtttatatacgggggcactgcgatttctcacttcttgaagaactgtttgtagcacaattacattcctgatggcagggtcctcaagaacatcaataagctgcctgggagtcgcaggctggaggccacagaagcccaggtccccggcctccaggcacttacaatctggtgcagtaacacattagtgtcgggcagcaagtagtgcggttgcgggcagacgctgctcgccgggtcctggggctgcggctccagggccggcccctcgtgcgcccctccacacgctgcgcacccgggcgcaccgcagccgatgtcgtctcgcaggtagtgctcgcgcacgatcttcatcacgccgcccgcccgggtcttttttaagaacgtcttggacttgagcatcttgcctcgccgcgcagaatcctaaccccagcagcgctcttccagcaaaaggcgtcaatctagaatac

SEQ ID NO: 14105 - RNA, 5048 nt, Homo sapiens
  source 1..5048: mol_type = other RNA
gctgggattacaggcatgagccaccgcacctagccggcaaacttttttaaatggttggcgggggtgggggaaatcaaatgagtaatgttttgtgacacatcaaaattataatgatgtgctgcataacttttggtcaacaatggccaaatatacgatgatgatcccgtaagattacaatggagctgaaaaattcctattgcctggggacacagccatggtaacatcatagtgaaattactttatgtagcctaagtatatagtgtttataaaagtctacagtagtgcacagtaatatcatggccttcacattcactaaccacttactgactcacccagagccagcttccagtcctgccaacttgttcatggtaaatgtcctaaataggtgtaccattttatatcttatatatatctatatatatatttttactgtaccttttctatgtttagatatgtttagatacacaaatacttagcactgtgttacaaccgcctacagtaatcagtacagtaatatgccatacaggtttgtaggttaggagcaataggctatcccatataggataccatagggtataccatctaggtttgtgtaactacatcatgattttcacacaatgatgaaattgccaagtgacatgtctcagaacatatccctgtcattaagtgacatatgactatatatgaaacttaacaaatcaggccttgttgaaacacagtcatgttgatttgtttacatattgtatatggctccttacacactatcaacggcagagttgtgtactatagttgcaatacagaccatagccaacaaagtctaaaatgttctagcacttcacagaaaaggttttttgactcctactctactgtttcagtgtcactgacccattttacctggaccaaagactactcaagtctattttcctccaactgacacaagtttctgcctcagtgtatggaggttttcctcagtaataggaaactggaaaaattagtcaacatttattgagtgcctaaatgactacctatttagtatacctgctgatttacttggcaggcttttctcactatactgcaagctccttgaaggcagagataatttacttgagtggaacctggcacaacgtaagtgctttagaaattgaataagccaagtaaaatgttttaaggcaaccctatcccaaaatattcctgaagatattaatttaatcattactaatctctgtgattagcaagggaagtagtcagtctggcacaccaaattttattaataatacttattttaatctgttccctttagtatgtctttatacagttcccctcgtgtatatacactgatataactacaatttaaaagccactaattaatctgttttttattttgtaagtaacaagatatagacatttgaatgccaatgtcttattctggagagacactggagctgaagttcaacaatgatcacacttattacctggcaataaaaacacaaccatctttccagtcaggtcaaaatatcctactttttgcctttctaccaattcccaaacattcacagtttttcaaggaccactaataaaatacaggaagcttttaaagacagtaagagaacacctagtgtaagttaggtgaattaaagatggcaaaggagattacatcctcaacactgacagcttccaagacttagaaaagagattgttccttgcttctaaaattgttctattttcctctgtaggaaaatgaaagttttttcttacaaatattaaataatcaaagtacttacgcaaaattaatctgctcctcaatgagatgagcactccatttaaatgatctttacagatccctgaagttgctgtcctgtcactgtatttaagtgatggatattcaattgaattattctgcataaataattctgttcaacccagaagtatagtagtatgatgggtcagatacagtcaactgttcaataaaaatgcagatgtctgaaattattaaaatgtacttaaaagtaacaaactgtatcacacacttaggcttagaagtgttctttcaagttttttcttttaaaaaagaaaccagtctttgaagatttttgttgaatatagctattttccaagcttcatcttctttttctttggtccattaaggtccatgtttgaagtatcagtaggaatgcttattcctggtatctgtggttctaccagggacattcggatcttctgatgttgaagattagatgagtctaacatgattttcactttaactttatcaaatacatggaacactgtatcttctattttaagtgagggtatctcatcatcataaataagctgtgggtttggtttgtccttttcttcaaaaaagactgtcccttctaaaccatactttggaattaataccacaatggcattctttcttacaaataaaatataggcttcttcacttactattcctttgcttttgaagaataactgggtatgaaaagccactgatgcacgttgggcatattgagccattttgtgccggaaatttagatttttacatatatctgcaagcttgtgtttgtctgtcaactctggataagtacagtcagccccaatagccacagccaaaagccgatgaacaatgacatctgcgtatcttctaatgggtgaagtaaaatgtgtgtatattggagacgctaagccatagtgatgaaaatcattatccattccagaacagaagtacacagcttgcatcatacagcgagtggctaatattctcaacagagtgtttagatatggaaaagtaggagattcggcctgatccaaagactcagccaaagacttggctgtatcagtcttaatttccaaattccttgacctggctgccttaacaagaatttcataatttgatggaggtggagcaggatgttttcgaagcagagcatgttcagaaaattcctcatgaattttttttgcaacagaaatattggcaagtaacataaattcttcaaccatggaatttgtttccctaagttccttggtctgcagatctataggatcgtgagtttcactgtccatgtggaatcgaacttcaggagaggatagagtcaaagcccctttttcaatccttcttttcttcagaattttggctagtttattcagtccacggagactagtggtaatatcatcattcatgtttgctgaatcaattctcaactgagcttcagcatacgtcagagatgcctttgaattaataacacttttggtaaacttcgtttttaagatttcagcattgtgattcatttcccaaatacatgaaaatgccagcctgtccacgtcacattttaaggaacacaagttagagctaagcaactctggaaccatgtcaatcctcttttcacaaagatacacagttgttcctcttctggctgattcttgatccaaggcatttcctggcctaataaaatggctcacatcagcaatatgaacaccaacctccaaatttccattttcgagttctcgacaatgtagagcatcgtctatatcagtacatcctggtgggtctacactacaaatacacagatgcctcaggtcttctcggtttttcatgtccttttcagtaatgctccagggcatctttggcagaaaactaagaacagcctgtgaaaaaggctgatggggaacatcgtgttcaagtaacaaaacttctgtttcagtctctttctctccaacatcacctaaatttctcacaaagtgtccatttggatatctggaatttctgggccaaccatcaatagcaacaataattctccgtccttctaatgtggaagcctgtctggtttctatgcgaattcgagggattctcttatcagcaggtgtaaagagatgtcttcttgactccttaatgtcagacttggaaagcatgccacaatatggtctccaattcctttttattattcctacaactctacctgtaggcttcaacattttctcgcttacagcagtcttaagcattcgttctgtctcttcttctttctccacatcttcttcattttgaccttcatcatgtaaaaccacagaagatggtgctacccactgactcttggggagaagctccacagccacaatatcttcgtgaacagctctgtttaaatgtttaagtccctgtaagattatctctttattttcttcattgtcgccatgaatccatactgtagcttccaagtaattttccctgctagctctaaatgttccttgaaggtatgtaccagattttatgccttgctgtagcttacttaagggaagatgctctgaaaatattatttttccactttctatttcattcccttcttcagacaaacaagcaagacgatctatgagttcggggttagcagttaggctctttacatattcttcacaagtgaaagctggtattccttcttctatggctttctctttgtttctcctgtcatttgttatgaagataacttgcagctggttgtctgctgacatttttttcaaatgttcattgtaccattttgctgctactcgaatcgctctatcattcctgtcattagcattttctccctgttcttgttctacataggtttctctatggtgctcattagtgaaagtatagaaatgcttctcttggttattagtcacatctcggatgcgtttatatacgggggcactgcgatttctcacttcttgaagaactgtttgtagcacaattacattcctgatggcagggtcctcaagaacatcaatctggtgcagtaacacattagtgtcgggcagcaagtagtgcggttgcgggcagacgctgctcgccgggtcctggggctgcggctccagggccggcccctcgtgcgcccctccacacgctgcgcacccgggcgcaccgcagccgatgtcgtctcgcaggtagtgctcgcgcacgatcttcatcacgccgcccgcccgggtcttttttaagaacgtcttggacttgagcatcttgcctcgccgcgcagaatcctaaccccagcagcgctcttccagcaaaaggcgtcaatctagaatac

SEQ ID NO: 14106 - RNA, 4890 nt, Homo sapiens
  source 1..4890: mol_type = other RNA
gctgggattacaggcatgagccaccgcacctagccggcaaacttttttaaatggttggcgggggtgggggaaatcaaatgagtaatgttttgtgacacatcaaaattataatgatgtgctgcataacttttggtcaacaatggccaaatatacgatgatgatcccgtaagattacaatggagctgaaaaattcctattgcctggggacacagccatggtaacatcatagtgaaattactttatgtagcctaagtatatagtgtttataaaagtctacagtagtgcacagtaatatcatggccttcacattcactaaccacttactgactcacccagagccagcttccagtcctgccaacttgttcatggtaaatgtcctaaataggtgtaccattttatatcttatatatatctatatatatatttttactgtaccttttctatgtttagatatgtttagatacacaaatacttagcactgtgttacaaccgcctacagtaatcagtacagtaatatgccatacaggtttgtaggttaggagcaataggctatcccatataggataccatagggtataccatctaggtttgtgtaactacatcatgattttcacacaatgatgaaattgccaagtgacatgtctcagaacatatccctgtcattaagtgacatatgactatatatgaaacttaacaaatcaggccttgttgaaacacagtcatgttgatttgtttacatattgtatatggctccttacacactatcaacggcagagttgtgtactatagttgcaatacagaccatagccaacaaagtctaaaatgttctagcacttcacagaaaaggttttttgactcctactctactgtttcagtgtcactgacccattttacctggaccaaagactactcaagtctattttcctccaactgacacaagtttctgcctcagtgtatggaggttttcctcagtaataggaaactggaaaaattagtcaacatttattgagtgcctaaatgactacctatttagtatacctgctgatttacttggcaggcttttctcactatactgcaagctccttgaaggcagagataatttacttgagtggaacctggcacaacgtaagtgctttagaaattgaataagccaagtaaaatgttttaaggcaaccctatcccaaaatattcctgaagatattaatttaatcattactaatctctgtgattagcaagggaagtagtcagtctggcacaccaaattttattaataatacttattttaatctgttccctttagtatgtctttatacagttcccctcgtgtatatacactgatataactacaatttaaaagccactaattaatctgttttttattttgtaagtaacaagatatagacatttgaatgccaatgtcttattctggagagacactggagctgaagttcaacaatgatcacacttattacctggcaataaaaacacaaccatctttccagtcaggtcaaaatatcctactttttgcctttctaccaattcccaaacattcacagtttttcaaggaccactaataaaatacaggaagcttttaaagacagtaagagaacacctagtgtaagttaggtgaattaaagatggcaaaggagattacatcctcaacactgacagcttccaagacttagaaaagagattgttccttgcttctaaaattgttctattttcctctgtaggaaaatgaaagttttttcttacaaatattaaataatcaaagtacttacgcaaaattaatctgctcctcaatgagatgagcactccatttaaatgatctttacagatccctgaagttgctgtcctgtcactgtatttaagtgatggatattcaattgaattattctgcataaataattctgttcaacccagaagtatagtagtatgatgggtcagatacagtcaactgttcaataaaaatgcagatgtctgaaattattaaaatgtacttaaaagtaacaaactgtatcacacacttaggcttagaagtgttctttcaagttttttcttttaaaaaagaaaccagtctttgaagatttttgttgaatatagctattttccaagcttcatcttctttttctttggtccattaaggtccatgtttgaagtatcagtaggaatgcttattcctggtatctgtggttctaccagggacattcggatcttctgatgttgaagattagatgagtctaacatgattttcactttaactttatcaaatacatggaacactgtatcttctattttaagtgagggtatctcatcatcataaataagctgtgggtttggtttgtccttttcttcaaaaaagactgtcccttctaaaccatactttggaattaataccacaatggcattctttcttacaaataaaatataggcttcttcacttactattcctttgcttttgaagaataactgggtatgaaaagccactgatgcacgttgggcatattgagccattttgtgccggaaatttagatttttacatatatctgcaagcttgtgtttgtctgtcaactctggataagtacagtcagccccaatagccacagccaaaagccgatgaacaatgacatctgcgtatcttctaatgggtgaagtaaaatgtgtgtatattggagacgctaagccatagtgatgaaaatcattatccattccagaacagaagtacacagcttgcatcatacagcgagtggctaatattctcaacagagtgtttagatatggaaaagtaggagattcggcctgatccaaagactcagccaaagacttggctgtatcagtcttaatttccaaattccttgacctggctgccttaacaagaatttcataatttgatggaggtggagcaggatgttttcgaagcagagcatgttcagaaaattcctcatgaattttttttgcaacagaaatattggcaagtaacataaattcttcaaccatggaatttgtttccctaagttccttggtctgcagatctataggatcgtgagtttcactgtccatgtggaatcgaacttcaggagaggatagagtcaaagcccctttttcaatccttcttttcttcagaattttggctagtttattcagtccacggagactagtggtaatatcatcattcatgtttgctgaatcaattctcaactgagcttcagcatacgtcagagatgcctttgaattaataacacttttggtaaacttcgtttttaagatttcagcattgtgattcatttcccaaatacatgaaaatgccagcctgtccacgtcacattttaaggaacacaagttagagctaagcaactctggaaccatgtcaatcctcttttcacaaagatacacagttgttcctcttctggctgattcttgatccaaggcatttcctggcctaataaaatggctcacatcagcaatatgaacaccaacctccaaatttccattttcgagttctcgacaatgtagagcatcgtctatatcagtacatcctggtgggtctacactacaaatacacagatgcctcaggtcttctcggtttttcatgtccttttcagtaatgctccagggcatctttggcagaaaactaagaacagcctgtgaaaaaggctgatggggaacatcgtgttcaagtaacaaaacttctgtttcagtctctttctctccaacatcacctaaatttctcacaaagtgtccatttggatatctggaatttctgggccaaccatcaatagcaacaataattctccgtccttctaatgtggaagcctgtctggtttctatgcgaattcgagggattctcttatcagcaggtgtaaagagatgtcttcttgactccttaatgtcagacttggaaagcatgccacaatatggtctccaattcctttttattattcctacaactctacctgtaggcttcaacattttctcgcttacagcagtcttaagcattcgttctgtctcttcttctttctccacatcttcttcattttgaccttcatcatgtaaaaccacagaagatggtgctacccactgactcttggggagaagctccacagccacaatatcttcgtgaacagctctgtttaaatgtttaagtccctgtaagattatctctttattttcttcattgtcgccatgaatccatactgtagcttccaagtaattttccctgctagctctaaatgttccttgaaggtatgtaccagattttatgccttgctgtagcttacttaagggaagatgctctgaaaatattatttttccactttctatttcattcccttcttcagacaaacaagcaagacgatctatgagttcggggttagcagttaggctctttacatattcttcacaagtgaaagctggtattccttcttctatggctttctctttgtttctcctgtcatttgttatgaagataacttgcagctggttgtctgctgacatttttttcaaatgttcattgtaccattttgctgctactcgaatcgctctatcattcctgtcattagcattttctccctgttcttgttctacataggtttctctggtgcagtaacacattagtgtcgggcagcaagtagtgcggttgcgggcagacgctgctcgccgggtcctggggctgcggctccagggccggcccctcgtgcgcccctccacacgctgcgcacccgggcgcaccgcagccgatgtcgtctcgcaggtagtgctcgcgcacgatcttcatcacgccgcccgcccgggtcttttttaagaacgtcttggacttgagcatcttgcctcgccgcgcagaatcctaaccccagcagcgctcttccagcaaaaggcgtcaatctagaatac

SEQ ID NO: 14107 - RNA, 2683 nt, Homo sapiens
  source 1..2683: mol_type = other RNA
gctgggattacaggcatgagccaccgcacctgctcacagcatataatttttcctctgaggactgaggaaagaatgaatgccttgggcatgacaagaagcagccctgcttcctctggagctctgcctcaaagggaacaagtcccaccacttccctgaccaggccctggcatcatgggagcaatcccattctctggcctggagcattctataatgctggccacatgcagaaacattacaagcaaaacaatgccagttgctatgggcacagagttggagagaagtatttccaaatattcaagaggatgctggggtgggtcgaatgggacaaattctgcaagttagaagcactaaatgtcctccatccagttaggtgacactccttgctgatttcttagcgcaaggtaggaagggccttgcagggatctgtctctgacactcaagatggcacaaaagcacatgggaaaacgtctttcggtcttttaaatcacagttgtctcattcaccctcagtgatctccgtccaagaggcagcaccatttagtttctgatcgtcaaggtgtttagcatcttttagaatatcatccaaattcatgacttcttggttcagatcctgaaactctttatactgctctttatgtggttctaatgcaagtaaaagcccattaaaagcatcctctaagcttccatctagaaaggatctgcagccttcagattctccaccaacagaaccctcagagagcagcctgtctgtggccattggcacctctgcagatgtgagcctcttgaccagctgctttgtgatgtttccttccgaagtgtccagttccacaggcttgagctcagaggcctcctcagactcttgcagaagtgcttctgcaacatcattctcaaggaacaggtgctcagccccagcacctgaggactgtcggcggcaagcctcagatggggccgaggcaggttttctgggctcctctgggtcttcctccttcaggtgtgactttggctcttggccttctcccagggagttcctggaagatgctgagctggtgtcatccataccctcattctgggaggccaagctgctgaggttaaactccgcaggggtgatggtaatttctggatttgttgagttggaaggggagcctgttgagtgggaggtgagggcgcagtccccgttgggcaggtcactgaagctgagcgacagtggcattttctcctcggctgcctttccattttcaaagatgtcatcaggtagatttgaaaagaaggagtggtctttgaaggtgggcgtttccggggtaccctggctgtacatggacattctcctctgaagggctgctgccttgttcccagcgcctgaggatgcggtcatgtcctccacgtcaaatggataccaggtgatttccaggttcagtttgatggtaccaaggtcattgatgtcgacagccactacctgaggtcgggctgcaaacagctctttggtctcacaggtcacgctacctaccaggatgtgagttgctagccctttgagctccgtgaccttgatggagatgaacccaactatcaggggcagaaaaactgtttcttctccatcccagctctgcttgccatttacttctattttgcctttcagtttccaccgctgccggccatacttcatgaaaatttcatattgatctccaggacagaggcgtgcaaagccagccagacctttcatcttgatggagaattctcccagcagattctctagctccacttcaatggtgcacatattctctgtgtactccttgaagctccgattgatctctgtcagactctcccgggcagctttgctggcaggggatgttgcgaaggcttgcttcattttgctggcaccatcctggaggcgtcgctggatacaataagcttcatagagttcatctaccttacttatatgaaactccaggcgtctcatgtatctttcaattgttttaatttgcttgtctaggtcatacagtacacccaggcgagagtttcttttcatatcttttaactgagctgtcaacttgtccagctccgtctggtgaacctccagatattcatcaagtccatttttcaaggccctgtagacttcttccacccttttaggctgaggctctttggggggattgttgtttttgtggcctaaattgtgcattttcttcagtttggcctgaggcttcttgagagcggaggaattttcaatgaaggagttacacctggatcgcctttcctggaggccgctgaaacccgcaaaggactggcttctaatgatcccattgggccctccaggcgaaaaagactgggatcctaccaacatgatttccgggagtctggtcggtagtccattgtcttagcaggtgacttcaatccagagagggggacaggctagcaggaaaaagggtaaatagttactgcccagattgaagactccaaagtgggcagacaacaaatcggtatgtttgcagagtgtcgacaattgccctttaaagactcaaagaaagaaaagctaaaaaaaacaacagcagcagaactctctggtagtacatccagatgtaatggaaagaccaatttcactagaccttcctcaaagctacgcgaagcagctcagcaaggaaggcagtttgagcgagttacttccccagagagagaaggacaaacagcct

SEQ ID NO: 14108 - RNA, 2716 nt, Homo sapiens
  source 1..2716: mol_type = other RNA
gctgggattacaggcatgagccaccgcacctgctcacagcatataatttttcctctgaggactgaggaaagaatgaatgccttgggcatgacaagaagcagccctgcttcctctggagctctgcctcaaagggaacaagtcccaccacttccctgaccaggccctggcatcatgggagcaatcccattctctggcctggagcattctataatgctggccacatgcagaaacattacaagcaaaacaatgccagttgctatgggcacagagttggagagaagtatttccaaatattcaagaggatgctggggtgggtcgaatgggacaaattctgcaagttagaagcactaaatgtcctccatccagttaggtgacactccttgctgatttcttagcgcaaggtaggaagggccttgcagggatctgtctctgacactcaagatggcacaaaagcacatgggaaaacgtctttcggtcttttaaatcacagttgtctcattcaccctcagtgatctccgtccaagaggcagcaccatttagtttctgatcgtcaaggtgtttagcatcttttagaatatcatccaaattcatgacttcttggttcagatcctgaaactctttatactgctctttatgtggttctaatgcaagtaaaagcccattaaaagcatcctctaagcttccatctagaaaggatctgcagccttcagattctccaccaacagaaccctcagagagcagcctgtctgtggccattggcacctctgcagatgtgagcctcttgaccagctgctttgtgatgtttccttccgaagtgtccagttccacaggcttgagctcagaggcctcctcagactcttgcagaagtgcttctgcaacatcattctcaaggaacaggtgctcagccccagcacctgaggactgtcggcggcaagcctcagatggggccgaggcaggttttctgggctcctctgggtcttcctccttcaggtgtgactttggctcttggccttctcccagggagttcctggaagatgctgagctggtgtcatccataccctcattctgggaggccaagctgctgaggttaaactccgcaggggtgatggtaatttctggatttgttgagttggaaggggagcctgttgagtgggaggtgagggcgcagtccccgttgggcaggtcactgaagctgagcgacagtggcattttctcctcggctgcctttccattttcaaagatgtcatcaggtagatttgaaaagaaggagtggtctttgaaggtgggcgtttccggggtaccctggctgtacatggacattctcctctgaagggctgctgccttgttcccagcgcctgaggatgcggtcatgtcctccacgtcaaatggataccaggtgatttccaggttcagtttgatggtaccaaggtcattgatgtcgacagccactacctgaggtcgggctgcaaacagctctttggtctcacaggtcacgctacctaccaggatgtgagttgctagccctttgagctccgtgaccttgatggagatgaacccaactatcaggggcagaaaaactgtttcttctccatcccagctctgcttgccatttacttctattttgcctttcagtttccaccgctgccggccatacttcatgaaaatttcatattgatctccaggacagaggcgtgcaaagccagccagacctttcatcttgatggagaattctcccagcagattctctagctccacttcaatggtgcacatattctctgtgtactccttgaagctccgattgatctctgtcagactctcccgggcagctttgctggcaggggatgttgcgaaggcttgcttcattttgctggcaccatcctggaggcgtcgctggatacaataagcttcatagagttcatctaccttacttatatgaaactccaggcgtctcatgtatctttcaattgttttaatttgcttgtctaggtcatacagtacacccaggcgagagtttcttttcatatcttttaactgagctgtcaacttgtccagctccgtctggtgaacctccagatattcatcaagtccatttttcaaggccctgtagacttcttccacccttttaggctgaggctctttggggggattgttgtttttgtggcctaaattgtgcattttcttcagtttggcctgaggcttcttgagagcggaggaattttcaatgaaggagttacacctggatcgcctttcctggaggccgctgaaacccgcaaaggactggcttctaatgatcccattgggccctccaggcgaaaaagactgggatcctaccaacatgatttccgggagtctggtcggtagtcctaacgacgacggctccttgtcatgtcaggggcacactcagggttctctggcatataaaagcctccgcaccaatgcaatgcccggagctgcccgcacctccggctttgcagacagcctgagctggctcacttgggtgaaggggaccccgggaggaagtcgggtggacgcgagctgtccccagcgccggctgccctgccgcgtccgctcgcagcagctgcggcgcgcggggtgaagttgcggggctggcgggcgcgagggtggcggagcgcggagctagagcggcggagcgggcggaggggcgggagccgtgaggagggggaggcgcggcgcgggggccggcggcgtcacttgt

SEQ ID NO: 14109 - RNA, 2724 nt, Homo sapiens
  source 1..2724: mol_type = other RNA
gctgggattacaggcatgagccaccgcacctgctcacagcatataatttttcctctgaggactgaggaaagaatgaatgccttgggcatgacaagaagcagccctgcttcctctggagctctgcctcaaagggaacaagtcccaccacttccctgaccaggccctggcatcatgggagcaatcccattctctggcctggagcattctataatgctggccacatgcagaaacattacaagcaaaacaatgccagttgctatgggcacagagttggagagaagtatttccaaatattcaagaggatgctggggtgggtcgaatgggacaaattctgcaagttagaagcactaaatgtcctccatccagttaggtgacactccttgctgatttcttagcgcaaggtaggaagggccttgcagggatctgtctctgacactcaagatggcacaaaagcacatgggaaaacgtctttcggtcttttaaatcacagttgtctcattcaccctcagtgatctccgtccaagaggcagcaccatttagtttctgatcgtcaaggtgtttagcatcttttagaatatcatccaaattcatgacttcttggttcagatcctgaaactctttatactgctctttatgtggttctaatgcaagtaaaagcccattaaaagcatcctctaagcttccatctagaaaggatctgcagccttcagattctccaccaacagaaccctcagagagcagcctgtctgtggccattggcacctctgcagatgtgagcctcttgaccagctgctttgtgatgtttccttccgaagtgtccagttccacaggcttgagctcagaggcctcctcagactcttgcagaagtgcttctgcaacatcattctcaaggaacaggtgctcagccccagcacctgaggactgtcggcggcaagcctcagatggggccgaggcaggttttctgggctcctctgggtcttcctccttcaggtgtgactttggctcttggccttctcccagggagttcctggaagatgctgagctggtgtcatccataccctcattctgggaggccaagctgctgaggttaaactccgcaggggtgatggtaatttctggatttgttgagttggaaggggagcctgttgagtgggaggtgagggcgcagtccccgttgggcaggtcactgaagctgagcgacagtggcattttctcctcggctgcctttccattttcaaagatgtcatcaggtagatttgaaaagaaggagtggtctttgaaggtgggcgtttccggggtaccctggctgtacatggacattctcctctgaagggctgctgccttgttcccagcgcctgaggatgcggtcatgtcctccacgtcaaatggataccaggtgatttccaggttcagtttgatggtaccaaggtcattgatgtcgacagccactacctgaggtcgggctgcaaacagctctttggtctcacaggtcacgctacctaccaggatgtgagttgctagccctttgagctccgtgaccttgatggagatgaacccaactatcaggggcagaaaaactgtttcttctccatcccagctctgcttgccatttacttctattttgcctttcagtttccaccgctgccggccatacttcatgaaaatttcatattgatctccaggacagaggcgtgcaaagccagccagacctttcatcttgatggagaattctcccagcagattctctagctccacttcaatggtgcacatattctctgtgtactccttgaagctccgattgatctctgtcagactctcccgggcagctttgctggcaggggatgttgcgaaggcttgcttcattttgctggcaccatcctggaggcgtcgctggatacaataagcttcatagagttcatctaccttacttatatgaaactccaggcgtctcatgtatctttcaattgttttaatttgcttgtctaggtcatacagtacacccaggcgagagtttcttttcatatcttttaactgagctgtcaacttgtccagctccgtctggtgaacctccagatattcatcaagtccatttttcaaggccctgtagacttcttccacccttttaggctgaggctctttggggggattgttgtttttgtggcctaaattgtgcattttcttcagtttggcctgaggcttcttgagagcggaggaattttcaatgaaggagttacacctggatcgcctttcctggaggccgctgaaacccgcaaaggactggcttctaatgatcccattgggccctccaggcgaaaaagactgggatcctaccaacatgatttccgggagtctggtcggtagtccttcaccaaaaacatcatcctcttcatcgaccaggagctcctcagcatcaaaaaactgcatcttggagaggacaggcgcgagaagcagcaggcagcagccccggcagtctcagcagtcacactgccgaccgaggtgatttcctttccttgggttgcccaagccctctggagggcagcttccgcatctgccctgaagaaagcagtttcattcatatgaataggcttcttgagccttgtgaagagtgaatcccaggtggggtaattctcaccactgaggagaaagaattttttgaagagggctgcagatccggttggatatgaatacagatatcactcaaagtctgaatgcaatgaattctat

SEQ ID NO: 14110 - RNA, 2681 nt, Homo sapiens
  source 1..2681: mol_type = other RNA
gctgggattacaggcatgagccaccgcacctgctcacagcatataatttttcctctgaggactgaggaaagaatgaatgccttgggcatgacaagaagcagccctgcttcctctggagctctgcctcaaagggaacaagtcccaccacttccctgaccaggccctggcatcatgggagcaatcccattctctggcctggagcattctataatgctggccacatgcagaaacattacaagcaaaacaatgccagttgctatgggcacagagttggagagaagtatttccaaatattcaagaggatgctggggtgggtcgaatgggacaaattctgcaagttagaagcactaaatgtcctccatccagttaggtgacactccttgctgatttcttagcgcaaggtaggaagggccttgcagggatctgtctctgacactcaagatggcacaaaagcacatgggaaaacgtctttcggtcttttaaatcacagttgtctcattcaccctcagtgatctccgtccaagaggcagcaccatttagtttctgatcgtcaaggtgtttagcatcttttagaatatcatccaaattcatgacttcttggttcagatcctgaaactctttatactgctctttatgtggttctaatgcaagtaaaagcccattaaaagcatcctctaagcttccatctagaaaggatctgcagccttcagattctccaccaacagaaccctcagagagcagcctgtctgtggccattggcacctctgcagatgtgagcctcttgaccagctgctttgtgatgtttccttccgaagtgtccagttccacaggcttgagctcagaggcctcctcagactcttgcagaagtgcttctgcaacatcattctcaaggaacaggtgctcagccccagcacctgaggactgtcggcggcaagcctcagatggggccgaggcaggttttctgggctcctctgggtcttcctccttcaggtgtgactttggctcttggccttctcccagggagttcctggaagatgctgagctggtgtcatccataccctcattctgggaggccaagctgctgaggttaaactccgcaggggtgatggtaatttctggatttgttgagttggaaggggagcctgttgagtgggaggtgagggcgcagtccccgttgggcaggtcactgaagctgagcgacagtggcattttctcctcggctgcctttccattttcaaagatgtcatcaggtagatttgaaaagaaggagtggtctttgaaggtgggcgtttccggggtaccctggctgtacatggacattctcctctgaagggctgctgccttgttcccagcgcctgaggatgcggtcatgtcctccacgtcaaatggataccaggtgatttccaggttcagtttgatggtaccaaggtcattgatgtcgacagccactacctgaggtcgggctgcaaacagctctttggtctcacaggtcacgctacctaccaggatgtgagttgctagccctttgagctccgtgaccttgatggagatgaacccaactatcaggggcagaaaaactgtttcttctccatcccagctctgcttgccatttacttctattttgcctttcagtttccaccgctgccggccatacttcatgaaaatttcatattgatctccaggacagaggcgtgcaaagccagccagacctttcatcttgatggagaattctcccagcagattctctagctccacttcaatggtgcacatattctctgtgtactccttgaagctccgattgatctctgtcagactctcccgggcagctttgctggcaggggatgttgcgaaggcttgcttcattttgctggcaccatcctggaggcgtcgctggatacaataagcttcatagagttcatctaccttacttatatgaaactccaggcgtctcatgtatctttcaattgttttaatttgcttgtctaggtcatacagtacacccaggcgagagtttcttttcatatcttttaactgagctgtcaacttgtccagctccgtctggtgaacctccagatattcatcaagtccatttttcaaggccctgtagacttcttccacccttttaggctgaggctctttggggggattgttgtttttgtggcctaaattgtgcattttcttcagtttggcctgaggcttcttgagagcggaggaattttcaatgaaggagttacacctggatcgcctttcctggaggccgctgaaacccgcaaaggactggcttctaatgatcccattgggccctccaggcgaaaaagactgggatcctaccaacatgatttccgggagtctggtcggtagtcggttgagctggcgcctccggatcctgtccctccatggcctgtttctgatccagtgtaatcgcgaaggtaacaccatggtcccaacagagcggcctaaaacctgctcatggcaaaggaacaaaagggtcttgcagctatcctggaagttaagtccagacgtataaaaatgaaaaagaaaacttaacccccccctttttgttcttttcttaaaaaaaaaaaaaagagtatttgaggcttccgttgacttcttttatcttgtaacttgccttgcctttccttcccttaacttccgactggcccgaaggcagctgctgtgct

SEQ ID NO: 14111 - RNA, 585 nt, Homo sapiens
  source 1..585: mol_type = other RNA
gctgggattacaggcatgagccaccgcacctggccaaaaattctgatttatatttgtgttttgccttatctttctattggacagcacagcaccagaatatcaatctgtgcctttgaggagacagcgggaacagtacaagaggattcaggagcctcagcctgaatcagagacccgacaaatcgcagaatgtatctaccacttggtgagattctgtccacatttacttcacaatcatctacacagatctggtgacaggccactctgcataagcgctctgaaggctttaggcaggtactggcaagtctgggtttcaggcagacagcatgttagaacgagcaggacagggagtcacatctctcagcatttgcatctcacctactagtgtgtgccctggggtacccatccccatgaactttcgtccatttttttaaaatggaacgtttataccaaagaggtcgttgtgagggtcaggtgaaataccaaacgatgagaataagtgtctcataattgtgagagcagcttacatttcacatagtgactattacagacacttaacaaaatgctttacaggtgacaacttattta

SEQ ID NO: 14112 - RNA, 1868 nt, Homo sapiens
  source 1..1868: mol_type = other RNA
gctgggattacaggcatgagccaccgcacctggccaaatctcagctctatttgttagccttatgtcctgtgtatttcgtttcctcatctgaaaatgaagaaaatagacatactcatctctgactgttattctaaggattaagtgctatataaagcacagcaaataattttgccagatgcaatagaaattagtttcttgaggaatgtgtcaatatctagcaattttacataggcatttaccctttgaaccagaaacttcacttatagaaatctatcctaaagacacacagtcaaaaattcaagacgggcatggtggttcatggctgtaatcctagcactttaggagacagaggagagaggattgcctgagctcaggagtttaagaccagcctggctaaatggcgaaaccccgtgtctactaaaaatacagaaagttagcccggcatggtggcaggtgcctgtaatcccagctacttgggaggctgagtcagcgaggaggaaatctacaggcagatgggcctccaatgccctcccagctgccctgcccacaggaagcccaacaccagaatcacacaggagggaaaaccccttgatcagtctgttatcagttactagaaggtgtgccccattagggagggaggtgaccgggaggaggaaggagtggcagcaggcctgggctgtcagtctctttctcttgcccacccttctctcttggcttcagtcttcctcttataagtgggatggaggtagggtcaccagacctgggaaggctaaggaccggaagcctggaacttggagagctgaggcaacagagaggctgcgtgcagaagtgagccatcatcgcaggaagccggccagcaggcaggccagcatggggcccagcagggcaggcagggcccagggcagcggccgacccggggccccggactttatcaccgtgcgctgccccagctgctgcaggggcctgacattgtccttcatgctcactgtctgttccttgtcgtagtacagcttctgagagaatgccaggatctgttctctgtgaagctgaatgggctcccggaacacagtccagacgaccttctcatcgcaggtcggtgtggtgagtgagcccaggtagcggaagtagtgcctcagtttctcctccttggggagcaggtccaacaggctgctctctgccatcgtagtgctcatctcaggtttggggatattagacagtgcctccaccagtggctggaagccctcgttcacctgggttccagcctccaccagaaaggccagcaccgcaatttcgtcttcagggtcctgggcctctttcacattcctcgatgtccccttctctttctcatgtactatgtgcatctccatggcaaagtgctccccatcgaggctgtgctccgagcccttatatggcaagtcggaccagtgcaggtgcaactgtttggcctggtatggggcaggcagtcctcctccagaaatgctggccttgttctccagcaacatcatcactgagtgcccgttattttggacagtccacgtttgcttcttatcgtagccagagaagaagaagcgtcccagttttttgtccacctttgccttggtggtgacgatgttgatgggggactggcggtccttctggcagtttccaccccacttgactggcaccaagcaggggtagttggaggactcggcttgaacctcgtagcaccagtgtgactctgcactggccgatggccgcgccgcggagagggccaggagcgccagcagcatccgcatcttgcgggacagcaaagagtcctctgagccgggggtcgcgcaccgaggaggccgccgcgggtgcagcgatcctgccggcctgggttttatagc

SEQ ID NO: 14113 - RNA, 6579 nt, Homo sapiens
  source 1..6579: mol_type = other RNA
gctgggattacaggcatgagccaccgcacctggccaatgtatcttggttgatttcttatgttacttgatctctgtaacatttaacattgttaactacttaacaatatagtcttggttttctcccaactctaagggtagttattcttctgtttaagggatcttctgattaaagtttctacatatcatcttaaatctctgaaaaatctgaaatcacttcagtatgaagttttccctaaggtccagccttttctcttttcacagcaagtcaagagatctagtgatagaaaatcttttaaattatgtgaagctgattagtgacacatagaggctttgcctaagcagaggtggggcagctgtgtcaatgatgcagctatgcgggggctgagatggactctaggagctgttccctgagattgagagctcatcacaatttctccacatctgtagaggctgcagaagaactgaaggagcagctgaggtcagtgcctctttacagctcttatgttcacaacacaatcagagttgtttattctggcattcaacatggtctgactctgctgaaacatctcctttctaaggctttccagaagggctgtctaggaaaaggaggaaatggagttggtgctgtgtgacttttaatgggataatccaacagcaagtgattagtcacctatagaatctaaagctaagcaattaggatttggctttattttcactaacttatgtggatcctcagtgctctacctttagacactgacaagaagaaaaagcatacatttgttaagctgggtccctgtagcttgtgtggaggaaatggtctcactgtgatgttgtaagctgggatcagagacccaggcactaattcagattcttctgcttgatgatgttgtggattcactgtagtgagtttggtccaagaaccagaagaagcttaatatctccaaacattctcttaaatggaagcattaagagcagacattaagtttttcttgagcactgatgtagccctaaggataaaaaagctgtagtgtggaattcatttccacactttttatccagtgccgtattttgggcattgtcatcaaggacgctggaccatgggaagctgtgctgatatatacggttcatttacacttgctttgtggccatcatatttccaatgtgattctatattcttgagtaaataaactgggaactcaagctaatcttatacaagtgtatatgtgtaatcttgatacacctccattgtccacctgaaacaatacagcttataggtgtgttctgaaaactaaagttgttacaatttgtttataattaagtaatctttttaaagagttagaagaatgtaagtgcagcattaatatttacttgacttttgtttttaaagtacttcaccaaaagttcattcctgaaagctgagctacatctgggctacttcatgttgtggactatggaagatctggtttaaaacttattttcatcaccccgggtgagtcatttactcttacacaaagatgtcatgagaatgagatccctcaaaacagaaaaataaccacccttagagtcggaggaaaaaaaaagtttaggtctcttaggtgtgggtgcaatggtgatggtagtactggggaaggaagtagtggtactggtagttagcataatcttatgaaatagtcataggatttcatatttcccttaagcatttttcatttattccagagaaactgtcaaaaacccataccctcgcatataaaacattcaataacctaagaaaaaaggaacttcctcaacatgtagagtacgtatgaaaaagccagagctaatgtcatactcaatggtgaaaagactaaaagtttttctcctaagaacaaaaacaagacaaggatgtcctcttctgctacttttatacaacacagtactacacatttttgccagagcaagtgagtaagaaaaagaaagggtatccaaatcggaaaggaagaagcaaaactatctttattcacagatgatatgatttatatgtagaaaaccctaaagaatgcaccaaaaaactggttagaactaaatctgcataagtcgcaggatacaaaatcaacacaggaaaatcagttgtatttctatccattagcgatgaacaatttcaaaaggaaatgaaggaaactattccatttacagtagtatccaaaagaataaaatgcccacaaataactttaagaaagtgaaaggcttgtacactgaaaactaaaacactgctcaaagaaattaaagaagacataagtggaaagacagcctgtgttcatggattggaagacttaaaattgctaagatgacaacactccctaaagcaatatgagggttcaatgcactctgtaacaaaatctcaatggtgttttgggcagaaatggaaaaactgatcctaaaattcctatgaaatttcaagtaacccacaatggtgtgtgtgtgtatatatacatatggcatgtatatatatgccatatatatatacgtgccatatatatatatatggaagaacaaaattggaagactcacacttccccatttcaaaacttactgcaaagctacagtagtcaaaacagtgtggtactggcataaagacagacatatagaccaacagaagagagttgagagcccagaaataatccctcacatgtgtggtcaactgatttttgacaagggtgctaagatcattcaatgcagaaagaacatctcctcaacaaatggtgctgggaaaactggctatccacatgcaaaagaatgaagttgggcacttacctcataccgtatacaaaaattaacttgaaatggatcaaagtcctaaatttaataaataaaactgtaaaattcatagaagaaaacacaggagcaaatcttcatgactttgcatttggcaacatgaaaagcctaagcaacaaaagaaaaaatggataagctggacttaataaaaattaaagtctgtctgcatcaaaagatacagtcaaaagagtaaaaggacaacccacagaatgggagaaaatacttgcaaaccatctatctgataagggcttaatatccagactctatgaagaaaagacaaacaacccagttttaaaaataggcaaaggacttgaatagacatttctttaaagaagatacaaaatagacaataagcatatgaaaagatgctcaacatcattagtcattagagaaatacaaatcaaaaccacaatgagacaccacttaacagctaccaagatggctataattttttaaaaaataacaagtgttgccagggatatggaaaaactagaactcttgtagattgctggtgggaatgtaaaatggtgccttcactatggaaaacagtttggtagtttcccaaaaagttaagcatagaattactgtatgactcagaaattccactcctatgtatacatccaagagaactgaaacaacagataaacaaatagattattatatgtaaatgttcatagcagtatcattcacaatagcccattggctattaatgaaaacaatctaagtgcccatcatcagaggaatggataaacaaaatgtggtatatatccatacaatggaatattattcagtcataaaaaaggaatgaagttctgatacacactacaacacagatgaaccttgaaaatgtgctaagtgaaataagccagatacaaaaggtcaaatgttgtatggttccatgaatatgaactgcttagaactggcaaattcacagaaaggttaccaggggtaggggataggggaatggagttattgcttaatgagaagagtttatgtttggagtgatggaaaaatgttggaaatggatagtggtgatggttgcctaacattgtgaatgtaattaatgtcactgaatttacacttaaaatcattacaatggcaaattttatattttatcacacacacaaaaataggcaaaggtaaagtttctacagtctcatgaagaaaagattaaataaaaagcttagtcacacctgacttgtgtgacagtaaaattatccctggacttgaggtcagaagatcagagttaactctcgatctcttgaccttgtgatctgcctgccttggtctcccaaagtgctgggattacaggcatgagccaccatgcccggcccagagttaagtctcttattgggctcctggtttgcactcttgggcccacaagagttattctctatacagccaccagaaaaaaaaagaaagaaagaaagaaactaagtactcatctaaaaattatctaaaaaagaacaatgaaagaaaccagaagaaactaggaaaaaattaagaagaatgaagtaaaaattaattaactagggaataaaaattgtagtaagtagaataagtaaaaaagcttatactttgaaaatacctatagataaaacatttgcaagactgatcacaaaaaaagcaaacattgacaagattactatccagaaataagacataaactctgatataatacatactgatagaattctaggacaataaatagagcatgcaggtgtgtgacagcagatttgaaaacacagaggtactaaatggtttccatttagtatatggtgaccaaaattgaccaaagtagaagtggaaaactgaaaagaccaatttcagagatgaaattagaagagttatttgacgtttaatggcaaaaaccaccagggaagtttggataaactattacaaatatcctctcaaaaccattataagagatcaagagaaagtaagggaaattcccagggaaccaaatagaggtgaaaacaggaggagtaagctacagctgggaccgaagctctgaagtccagcttgccaacctcagtaacaaaggagtttagaatacagtgactgtggcaggacaagacatagtcccatgggactacataaagtagggagaggaactgagaccctgacatgaagctggggcaccagaaatgaaaaggtaaatcagaaaaaaaaaaaaaaaaaaaaatcttccaagaaagctcaggtgtttcagcaagggctctaggtgggctctgtgtgtttcttccctatcacattctcaagtcattccctcaagataactattatcctggattttgtgtttgtgtttacacagagttctgcttgattttaagtaaaaaattgtatactaaggtagtcttctgtgacttgagtttttcacttagtattgtgtttatgaaaaaatttaaaccctatgtttactgataaccacaaggaataacagacacaatatttaataaaaaaaggaacaaaatatcgaaaccatctatatactgtaatgtacctttaaaccaatgctagggaaaaacaaagggaaaacacaaaactgcaataaacttcatcttctctcccaggtttttcttgaacaattcccacccccattccctactatgtatccttaacttctttagacagtgaatgagaaattaatactaaaagccctcaaatgaaccctagggacatttcctgggttttcccttcttctcccctctccaaccgtgccgtgaagggcaagcccctcagccctaaaatctgaggaggcccagagtggtggctggggcagaggagtgggctacccctgcagagtagagacgtgtatagtgggggatatccactgggagccccagtcccaggtgaaagcacactggtgctcctgggcaaggaggcccggctgtccccacaatctcccgtggggaagcatcattggttggtcgactgcccatcttgctgcggttatagaaccaaactcgaaccacatccttctgcagctggaggcacccagcaatgtggctgatttgctggggtgtgggcttagggcaccgctggaagaatttctccaggctgtttccgattcgtcgctctctgcttgcccgtctccacttcccagactgttgcaggatcatctccattttgcataagcccagaaggttctctgcttccacttccttcagccactttttcagcagtggtcgcagcttccacatgttggcgacgcttagctgctgggcctcgaagcggcagatggtcgtctggctaagcaccttcccaaacagagctcccacagcgatccccacatcggcctgcgagtaccctaggctcaacctcttctgcctcaactccttggccaattgctgcaactctttcagtatgcccgagatgtcctctggcggcggcaacttcggaatgctccgcagggcaatgtagggccccgggagggcgccttcggaggggcgtcgcaaccagtcccctgcctcactagctccaagacggggcctgcagggtgctatccagccccggaattcgtgtggcaggggacccaggggaatcctccacacgtcagggcctgggcagatccctggcctgactgccggccagaccatcaccctgccaggggccgcctgggtgctcaaccaggtcagagtgtcaacccgcaggggcatcggccctctggggccgcccccaccactgcctggaagggggcagaagtggtttgagggcctgtgtccggccatgggtggaatggcacccgcagcggctctggtaggaact

SEQ ID NO: 14114 - RNA, 5722 nt, Homo sapiens
  source 1..5722: mol_type = other RNA
gctgggattacaggcatgagccaccgcacctggccacttggctgttctttacttgggttggttttattttgttgtttcctttttcttgacggaaatacttattcattccctcaacacattcatctgtgtgacaggcctggtgttgctgctgtgggtaagtgaagaagatgaagactgtatccacaaataagatttccttaccacattacagggcattaatttgtcactgaacagaactttgattatatctgacaaggttagatgtgcaggcatctcactgtcattcatttctacatagtctataattttggttttgattttaaacattttattattgaaatttcaaacacatacaaaagtagaaatattagaacaataagtctccatgaacaaaacactccacttaaattatcaacatgttgccaatttagtttccagctctctttgccaattatttcttttgctagaatattttaatccaaatgtgtctatcttcatttcatagtatgtatctcatatcatacgatcttttattttttataatcacactgacataatccctaaccaaattaatatatgtaaatatcatttaatatttagtccatgtccacacttccctcactgtctccaaaatggctttttatgttttgttcaaaccaggtccaagtaatgccaacatactgaatttagttgatatgtctctttaagtctcttttaatctgttaatggttgcccttccccttgtattttcatgctacctgttagttgaagaaatcaggtaatttgctctgtagaatttcacacattctggatctgtttggcttcttccttgtggtgccctttatagccagccctccatatgtgcagattcaaccaatctcaaatagaaaatactcaaaaaaaaacaataaaaataaaatacaataaaaataatgcaaattgaaaaatacagtataacaactatttacatagtatttacattgtgataggtataagtgatctaaagataatttaaagtatacaggaagatgtgagtaggtaatatgcaaatacatactatgccattttatacaagggacttgagcatcctcagattttaccatcagtggaggatcctggaaccaattccccatggataccaagggatgaccatatactgttcatctagtccctgtctgctttcagttcattattccagcaataaggctttgtagatggtggtgtggacttcctattgcattacgtcaggaagtgtgttgtctgatagacccatttttattaaggttaaaacagatcaaagggttcagaggtggccagtttgatagatccaccataaaaatctcgctataaaatatttcacctattagttgtagtacccattgaagatcatgttttctggacccattattccattaaggtctagaaaatggtgatttttctaatcctctaattccttctagatttattagacttcttcaaaaaagaaaaacccattcaaaaaacaaattttttttttgagacagggtctcactctgtcacccaggctggagtgcagtggcacgatctcagctcactgcaaactctgcctcttgggttcaagtgatcctcccacctcagcctgggactacaggtgtgtgccaccatgcctggctaaattttgtatttttagtacagacagggtttcaccatgttaaccaggttggtctcaaactcctggcctcaagtgatccacccaccttgtcctcccaaagtgctgggattacaggtgtgacccctgtgccaggccaaattcatttgaatttgatgaacttctggtgaccctgaaatttggttcacatgggaaaaggaaactaaatgacaatttttcctctgatttattgatttcaagaataatgagttgggctgggtgtggtggctcatacctgtaaccccagcacctttggaggccaaggagggaggatcacttgagcccagaagttcaagaccagcctgggcaacatagtgagaccctttctctaaaaaaaaaaaaaaaatttaggtggaagaatcacttgagcccaggaggaacagggtacagtgaactgtgcttgtaccactgcactccagcctgggggacaaagtgacaccctgtctcaaaaaaattatacattggtgctctagcatctttcataggttaccaaattatgcagccacaatcaagtaaactatcaaattattggtgggatcacatcaaaaactcaacttgaaacaactcctactggttgaagatatggcattttgagcatccaaaagtatactgacttatagaatgatgttttgtttctttcccacaggagttttatacacacacataaatatacacaacaatattaaattcctaggtggttaatttcttttaagccacatttttgatagtttctaattaattttaaactgtggtcagacaacagggattgtaagccttttgctttctggaattatgggaaaatcatttcctatttccctctaattcttcaacagctgtattactagtgacctcacattcatgaaattcatttttggcatgaaatttctaatgcagctcaagtgctgaagaacttcctacattcactacaatctaaattttacctagaataaattatgtttaataatttctgagaggtgacaggaggcatttctacatttattatgtctacagatcttccttttacgtgaattcactaatactaatgacaataataacaattacagataatatttacagaatacatgctatatgactgtgattcctccaagtattaactacttactccttgcaacaatcctattccacagtgtggcaggctgactctaaacaggccccccagtggtcctgtctccaggacttattcacactcttgtatcatcccgttctcttgagtgtggactatcctagtaacttacttctaccagtagaaggtgagggaatgttacttccatgattagattacacaagatggtaacttccatcttgctagcagactgtcctcccttttggcttgcatgccttgatgaagcaagcagccatgttgatgaggctattgtggccaggagctgcagtcagcgttcagccaacagccagctagaaactgagaatctcaatgcaacaggcctcacggaaatacattgggtaacaactatgttagtctggatgtggatccttccccagttgagccttcagatgagacctcagccctggctgaaatctgtagccttgcaagagaccctgaagcagaggacccaactaagtcatgcctatactcctgatccaaattataagatataattatatgttattttatgctactaagtctgtggtaatttattacgcagcaataaataactaatacatataagtactattattaccattttacaagtcagcaaaatgaggcacagaagcttagtatcttgtccaataaatcaaactggtaatcaagtggagaaagggagataatgacagataaggctaaagattttcctacattcattacattattctctcataggaatttgctgaagataaaccatgtttaaatggtgttggaaggcttttaaatcaacatattctttctctaatataaaatttattatgcttggaattgagcatgaaacacattttctcaaaaatgaattttctgatgttctgtaacatcatatacatttgaaggctttcttctattaaattccattatgaatcttctgatgctgagtaaggtgtgaatgctgtctaaaggccttcttacactccttacacttgtagggcttctcaccagtatgaattctctggtgttgagtaagaaatgaataaagtctaaaagccttaccacattccttacattcataaggtttctcaccagtgtgaatactctgatgttgggtaagttgtgagagcagtctaaaaggttttctacattccttacattcataaggtttctcaccagtgtgaatactttgatgctgagtaagttgtgagagcagtctaaaggcctttccacactcttcacattcatagggtctctcaccaatatgaatgctctggtgtgaaataagctgtgagtaactactaaaggtcttccaacattccatacattcatagggtttctcacgagtatgtattctctgatggcgaactagttgttgtcttaatctaaaagtcttcccacattccttacattcgtagggtttctcaccagtatgaatactctgatgaacagtaagttgttggcatattctaaaagcctttccacactccttacattcatagggtttctcaccaaaatgaattttctgatgtactctaaggtctggaccacatacgaaggctttcccacattccttacattcatagagcttttcagcagtatgaagtctctgatggcgtgtaaggtgtgtacactgtctaaaggtctttccacagtccttacattcatagggtttctcaccagtgtgaattctctgatgtcgagccagttgctgatgtactctaaaggcctttccacattccttacattcatagggtttttcacccgtatgaagtctctgatgttgagtaagttcttggagcactgtaaaggccttcccacactccttacattcatagggtttctcaccggtgtgaagtttgtgatgtcgaataagatgtgcacgctgtctaaaggcctgcccacattccttacacttataaggtttctcaccagtatgaattctcaggtgttgactaagtgttgagcgacgaataaaggtcttcctacactccttacactcatacaccttttctccattatgaacgatctgatactcagtaagaaaattgtgccttttgtaagtggtcattttttcagaggtaattttcacttgcccaaaatatccctcttgttgttccttttccccctcaatcttgcttttgcattcccaatcattcctaaaaatggaaccctgaaggctatagcttttaattctttccattatatcccactgaaatgaatatatttcataaatgtccttttctggagataaagtattggtcctgtatctggactccaaatcagggcagtatcttcttgtcccttccctcacaaccatcccaggttccttcctttcttcatccaataaggtaatcacatctggtttagaaatggaaggtcctagtgaaatgaagttgctgtagttctcccacattacatccctatataagtccctctgagcaggatccaggaattcccattcttcctgtgagaagtctatggccacatccctgaatgtcactgaaccatgggccatggttttagaactgcaaaaactggtcagtccttttcaagatttctctgttggagaactatggagtcctgataagccagagcctttcccgtatcagagcgaaaggccaggtacacgaagacggggctgggatctgtctccgagttccccgcagtttccatgggagggagctcgggtaaagctgtgcaatctgcagttcttcagactgcgtctttttgtttgggggccttcattcactccggggttcctgtatctaactcggagccattccgggccgctggacctgggcggctctgaagcgagaaggcagaggacgcaacagggcacccggcgcccagtcagcgccacaaactccacagctactgcctcctggctcacactgaggtctgcgccgcccccgcgc

SEQ ID NO: 14115 - RNA, 5440 nt, Homo sapiens
  source 1..5440: mol_type = other RNA
gctgggattacaggcatgagccaccgcacctggccacttggctgttctttacttgggttggttttattttgttgtttcctttttcttgacggaaatacttattcattccctcaacacattcatctgtgtgacaggcctggtgttgctgctgtgggtaagtgaagaagatgaagactgtatccacaaataagatttccttaccacattacagggcattaatttgtcactgaacagaactttgattatatctgacaaggttagatgtgcaggcatctcactgtcattcatttctacatagtctataattttggttttgattttaaacattttattattgaaatttcaaacacatacaaaagtagaaatattagaacaataagtctccatgaacaaaacactccacttaaattatcaacatgttgccaatttagtttccagctctctttgccaattatttcttttgctagaatattttaatccaaatgtgtctatcttcatttcatagtatgtatctcatatcatacgatcttttattttttataatcacactgacataatccctaaccaaattaatatatgtaaatatcatttaatatttagtccatgtccacacttccctcactgtctccaaaatggctttttatgttttgttcaaaccaggtccaagtaatgccaacatactgaatttagttgatatgtctctttaagtctcttttaatctgttaatggttgcccttccccttgtattttcatgctacctgttagttgaagaaatcaggtaatttgctctgtagaatttcacacattctggatctgtttggcttcttccttgtggtgccctttatagccagccctccatatgtgcagattcaaccaatctcaaatagaaaatactcaaaaaaaaacaataaaaataaaatacaataaaaataatgcaaattgaaaaatacagtataacaactatttacatagtatttacattgtgataggtataagtgatctaaagataatttaaagtatacaggaagatgtgagtaggtaatatgcaaatacatactatgccattttatacaagggacttgagcatcctcagattttaccatcagtggaggatcctggaaccaattccccatggataccaagggatgaccatatactgttcatctagtccctgtctgctttcagttcattattccagcaataaggctttgtagatggtggtgtggacttcctattgcattacgtcaggaagtgtgttgtctgatagacccatttttattaaggttaaaacagatcaaagggttcagaggtggccagtttgatagatccaccataaaaatctcgctataaaatatttcacctattagttgtagtacccattgaagatcatgttttctggacccattattccattaaggtctagaaaatggtgatttttctaatcctctaattccttctagatttattagacttcttcaaaaaagaaaaacccattcaaaaaacaaattttttttttgagacagggtctcactctgtcacccaggctggagtgcagtggcacgatctcagctcactgcaaactctgcctcttgggttcaagtgatcctcccacctcagcctgggactacaggtgtgtgccaccatgcctggctaaattttgtatttttagtacagacagggtttcaccatgttaaccaggttggtctcaaactcctggcctcaagtgatccacccaccttgtcctcccaaagtgctgggattacaggtgtgacccctgtgccaggccaaattcatttgaatttgatgaacttctggtgaccctgaaatttggttcacatgggaaaaggaaactaaatgacaatttttcctctgatttattgatttcaagaataatgagttgggctgggtgtggtggctcatacctgtaaccccagcacctttggaggccaaggagggaggatcacttgagcccagaagttcaagaccagcctgggcaacatagtgagaccctttctctaaaaaaaaaaaaaaaatttaggtggaagaatcacttgagcccaggaggaacagggtacagtgaactgtgcttgtaccactgcactccagcctgggggacaaagtgacaccctgtctcaaaaaaattatacattggtgctctagcatctttcataggttaccaaattatgcagccacaatcaagtaaactatcaaattattggtgggatcacatcaaaaactcaacttgaaacaactcctactggttgaagatatggcattttgagcatccaaaagtatactgacttatagaatgatgttttgtttctttcccacaggagttttatacacacacataaatatacacaacaatattaaattcctaggtggttaatttcttttaagccacatttttgatagtttctaattaattttaaactgtggtcagacaacagggattgtaagccttttgctttctggaattatgggaaaatcatttcctatttccctctaattcttcaacagctgtattactagtgacctcacattcatgaaattcatttttggcatgaaatttctaatgcagctcaagtgctgaagaacttcctacattcactacaatctaaattttacctagaataaattatgtttaataatttctgagaggtgacaggaggcatttctacatttattatgtctacagatcttccttttacgtgaattcactaatactaatgacaataataacaattacagataatatttacagaatacatgctatatgactgtgattcctccaagtattaactacttactccttgcaacaatcctattccacagtgtggcaggctgactctaaacaggccccccagtggtcctgtctccaggacttattcacactcttgtatcatcccgttctcttgagtgtggactatcctagtaacttacttctaccagtagaaggtgagggaatgttacttccatgattagattacacaagatggtaacttccatcttgctagcagactgtcctcccttttggcttgcatgccttgatgaagcaagcagccatgttgatgaggctattgtggccaggagctgcagtcagcgttcagccaacagccagctagaaactgagaatctcaatgcaacaggcctcacggaaatacattgggtaacaactatgttagtctggatgtggatccttccccagttgagccttcagatgagacctcagccctggctgaaatctgtagccttgcaagagaccctgaagcagaggacccaactaagtcatgcctatactcctgatccaaattataagatataattatatgttattttatgctactaagtctgtggtaatttattacgcagcaataaataactaatacatataagtactattattaccattttacaagtcagcaaaatgaggcacagaagcttagtatcttgtccaataaatcaaactggtaatcaagtggagaaagggagataatgacagataaggctaaagattttcctacattcattacattattctctcataggaatttgctgaagataaaccatgtttaaatggtgttggaaggcttttaaatcaacatattctttctctaatataaaatttattatgcttggaattgagcatgaaacacattttctcaaaaatgaattttctgatgttctgtaacatcatatacatttgaaggctttcttctattaaattccattatgaatcttctgatgctgagtaaggtgtgaatgctgtctaaaggccttcttacactccttacacttgtagggcttctcaccagtatgaattctctggtgttgagtaagaaatgaataaagtctaaaagccttaccacattccttacattcataaggtttctcaccagtgtgaatactctgatgttgggtaagttgtgagagcagtctaaaaggttttctacattccttacattcataaggtttctcaccagtgtgaatactttgatgctgagtaagttgtgagagcagtctaaaggcctttccacactcttcacattcatagggtctctcaccaatatgaatgctctggtgtgaaataagctgtgagtaactactaaaggtcttccaacattccatacattcatagggtttctcacgagtatgtattctctgatggcgaactagttgttgtcttaatctaaaagtcttcccacattccttacattcgtagggtttctcaccagtatgaatactctgatgaacagtaagttgttggcatattctaaaagcctttccacactccttacattcatagggtttctcaccaaaatgaattttctgatgtactctaaggtctggaccacatacgaaggctttcccacattccttacattcatagagcttttcagcagtatgaagtctctgatggcgtgtaaggtgtgtacactgtctaaaggtctttccacagtccttacattcatagggtttctcaccagtgtgaattctctgatgtcgagccagttgctgatgtactctaaaggcctttccacattccttacattcatagggtttttcacccgtatgaagtctctgatgttgagtaagttcttggagcactgtaaaggccttcccacactccttacattcatagggtttctcaccggtgtgaagtttgtgatgtcgaataagatgtgcacgctgtctaaaggcctgcccacattccttacacttataaggtttctcaccagtatgaattctcaggtgttgactaagtgttgagcgacgaataaaggtcttcctacactccttacactcatacaccttttctccattatgaacgatctgatactcagtaagaaaattgtgccttttgtaagtggtcattttttcagaggtaattttcacttgcccaaaatatccctcttgttgttccttttccccctcaatcttgcttttgcattcccaatcattcctaaaaatggaaccctgaaggctatagcttttaattctttccattatatcccactgaaatgaatatatttcataaatgtccttttctggagataaagtattggtcctgtatctggactccaaatcagggcagtatcttcttgtcccttccctcacaaccatcccaggttccttcctttcttcatccaataaggtaatcacatctggtttagaaatggaaggtcctagtgaaatgaagttgctgtagttctcccacattacatccctatataagtccctctgagcaggatccaggaattcccattcttcctgtgagaagtctatggccacatccctgaatgtcactgaaccatgggccatggttttagaactgcaaaaactggtcagtccttttcaagatttctctgttggagaactatggagtcctgataagccagagctctcggagccgacaccagcagcgaagccggaaagaact

SEQ ID NO: 14116 - RNA, 5443 nt, Homo sapiens
  source 1..5443: mol_type = other RNA
gctgggattacaggcatgagccaccgcacctggccacttggctgttctttacttgggttggttttattttgttgtttcctttttcttgacggaaatacttattcattccctcaacacattcatctgtgtgacaggcctggtgttgctgctgtgggtaagtgaagaagatgaagactgtatccacaaataagatttccttaccacattacagggcattaatttgtcactgaacagaactttgattatatctgacaaggttagatgtgcaggcatctcactgtcattcatttctacatagtctataattttggttttgattttaaacattttattattgaaatttcaaacacatacaaaagtagaaatattagaacaataagtctccatgaacaaaacactccacttaaattatcaacatgttgccaatttagtttccagctctctttgccaattatttcttttgctagaatattttaatccaaatgtgtctatcttcatttcatagtatgtatctcatatcatacgatcttttattttttataatcacactgacataatccctaaccaaattaatatatgtaaatatcatttaatatttagtccatgtccacacttccctcactgtctccaaaatggctttttatgttttgttcaaaccaggtccaagtaatgccaacatactgaatttagttgatatgtctctttaagtctcttttaatctgttaatggttgcccttccccttgtattttcatgctacctgttagttgaagaaatcaggtaatttgctctgtagaatttcacacattctggatctgtttggcttcttccttgtggtgccctttatagccagccctccatatgtgcagattcaaccaatctcaaatagaaaatactcaaaaaaaaacaataaaaataaaatacaataaaaataatgcaaattgaaaaatacagtataacaactatttacatagtatttacattgtgataggtataagtgatctaaagataatttaaagtatacaggaagatgtgagtaggtaatatgcaaatacatactatgccattttatacaagggacttgagcatcctcagattttaccatcagtggaggatcctggaaccaattccccatggataccaagggatgaccatatactgttcatctagtccctgtctgctttcagttcattattccagcaataaggctttgtagatggtggtgtggacttcctattgcattacgtcaggaagtgtgttgtctgatagacccatttttattaaggttaaaacagatcaaagggttcagaggtggccagtttgatagatccaccataaaaatctcgctataaaatatttcacctattagttgtagtacccattgaagatcatgttttctggacccattattccattaaggtctagaaaatggtgatttttctaatcctctaattccttctagatttattagacttcttcaaaaaagaaaaacccattcaaaaaacaaattttttttttgagacagggtctcactctgtcacccaggctggagtgcagtggcacgatctcagctcactgcaaactctgcctcttgggttcaagtgatcctcccacctcagcctgggactacaggtgtgtgccaccatgcctggctaaattttgtatttttagtacagacagggtttcaccatgttaaccaggttggtctcaaactcctggcctcaagtgatccacccaccttgtcctcccaaagtgctgggattacaggtgtgacccctgtgccaggccaaattcatttgaatttgatgaacttctggtgaccctgaaatttggttcacatgggaaaaggaaactaaatgacaatttttcctctgatttattgatttcaagaataatgagttgggctgggtgtggtggctcatacctgtaaccccagcacctttggaggccaaggagggaggatcacttgagcccagaagttcaagaccagcctgggcaacatagtgagaccctttctctaaaaaaaaaaaaaaaatttaggtggaagaatcacttgagcccaggaggaacagggtacagtgaactgtgcttgtaccactgcactccagcctgggggacaaagtgacaccctgtctcaaaaaaattatacattggtgctctagcatctttcataggttaccaaattatgcagccacaatcaagtaaactatcaaattattggtgggatcacatcaaaaactcaacttgaaacaactcctactggttgaagatatggcattttgagcatccaaaagtatactgacttatagaatgatgttttgtttctttcccacaggagttttatacacacacataaatatacacaacaatattaaattcctaggtggttaatttcttttaagccacatttttgatagtttctaattaattttaaactgtggtcagacaacagggattgtaagccttttgctttctggaattatgggaaaatcatttcctatttccctctaattcttcaacagctgtattactagtgacctcacattcatgaaattcatttttggcatgaaatttctaatgcagctcaagtgctgaagaacttcctacattcactacaatctaaattttacctagaataaattatgtttaataatttctgagaggtgacaggaggcatttctacatttattatgtctacagatcttccttttacgtgaattcactaatactaatgacaataataacaattacagataatatttacagaatacatgctatatgactgtgattcctccaagtattaactacttactccttgcaacaatcctattccacagtgtggcaggctgactctaaacaggccccccagtggtcctgtctccaggacttattcacactcttgtatcatcccgttctcttgagtgtggactatcctagtaacttacttctaccagtagaaggtgagggaatgttacttccatgattagattacacaagatggtaacttccatcttgctagcagactgtcctcccttttggcttgcatgccttgatgaagcaagcagccatgttgatgaggctattgtggccaggagctgcagtcagcgttcagccaacagccagctagaaactgagaatctcaatgcaacaggcctcacggaaatacattgggtaacaactatgttagtctggatgtggatccttccccagttgagccttcagatgagacctcagccctggctgaaatctgtagccttgcaagagaccctgaagcagaggacccaactaagtcatgcctatactcctgatccaaattataagatataattatatgttattttatgctactaagtctgtggtaatttattacgcagcaataaataactaatacatataagtactattattaccattttacaagtcagcaaaatgaggcacagaagcttagtatcttgtccaataaatcaaactggtaatcaagtggagaaagggagataatgacagataaggctaaagattttcctacattcattacattattctctcataggaatttgctgaagataaaccatgtttaaatggtgttggaaggcttttaaatcaacatattctttctctaatataaaatttattatgcttggaattgagcatgaaacacattttctcaaaaatgaattttctgatgttctgtaacatcatatacatttgaaggctttcttctattaaattccattatgaatcttctgatgctgagtaaggtgtgaatgctgtctaaaggccttcttacactccttacacttgtagggcttctcaccagtatgaattctctggtgttgagtaagaaatgaataaagtctaaaagccttaccacattccttacattcataaggtttctcaccagtgtgaatactctgatgttgggtaagttgtgagagcagtctaaaaggttttctacattccttacattcataaggtttctcaccagtgtgaatactttgatgctgagtaagttgtgagagcagtctaaaggcctttccacactcttcacattcatagggtctctcaccaatatgaatgctctggtgtgaaataagctgtgagtaactactaaaggtcttccaacattccatacattcatagggtttctcacgagtatgtattctctgatggcgaactagttgttgtcttaatctaaaagtcttcccacattccttacattcgtagggtttctcaccagtatgaatactctgatgaacagtaagttgttggcatattctaaaagcctttccacactccttacattcatagggtttctcaccaaaatgaattttctgatgtactctaaggtctggaccacatacgaaggctttcccacattccttacattcatagagcttttcagcagtatgaagtctctgatggcgtgtaaggtgtgtacactgtctaaaggtctttccacagtccttacattcatagggtttctcaccagtgtgaattctctgatgtcgagccagttgctgatgtactctaaaggcctttccacattccttacattcatagggtttttcacccgtatgaagtctctgatgttgagtaagttcttggagcactgtaaaggccttcccacactccttacattcatagggtttctcaccggtgtgaagtttgtgatgtcgaataagatgtgcacgctgtctaaaggcctgcccacattccttacacttataaggtttctcaccagtatgaattctcaggtgttgactaagtgttgagcgacgaataaaggtcttcctacactccttacactcatacaccttttctccattatgaacgatctgatactcagtaagaaaattgtgccttttgtaagtggtcattttttcagaggtaattttcacttgcccaaaatatccctcttgttgttccttttccccctcaatcttgcttttgcattcccaatcattcctaaaaatggaaccctgaaggctatagcttttaattctttccattatatcccactgaaatgaatatatttcataaatgtccttttctggagataaagtattggtcctgtatctggactccaaatcagggcagtatcttcttgtcccttccctcacaaccatcccaggttccttcctttcttcatccaataaggtaatcacatctggtttagaaatggaaggtcctgctagtgaaatgaagttgctgtagttctcccacattacatccctatataagtccctctgagcaggatccaggaattcccattcttcctgtgagaagtctatggccacatccctgaatgtcactgaaccatgggccatggttttagaactgcaaaaactggtcagtccttttcaagatttctctgttggagaactatggagtcctgataagccagagctctcggagccgacaccagcagcgaagccggaaagaact

SEQ ID NO: 14117 - RNA, 5175 nt, Homo sapiens
  source 1..5175: mol_type = other RNA
gctgggattacaggcatgagccaccgcacctggccacttggctgttctttacttgggttggttttattttgttgtttcctttttcttgacggaaatacttattcattccctcaacacattcatctgtgtgacaggcctggtgttgctgctgtgggtaagtgaagaagatgaagactgtatccacaaataagatttccttaccacattacagggcattaatttgtcactgaacagaactttgattatatctgacaaggttagatgtgcaggcatctcactgtcattcatttctacatagtctataattttggttttgattttaaacattttattattgaaatttcaaacacatacaaaagtagaaatattagaacaataagtctccatgaacaaaacactccacttaaattatcaacatgttgccaatttagtttccagctctctttgccaattatttcttttgctagaatattttaatccaaatgtgtctatcttcatttcatagtatgtatctcatatcatacgatcttttattttttataatcacactgacataatccctaaccaaattaatatatgtaaatatcatttaatatttagtccatgtccacacttccctcactgtctccaaaatggctttttatgttttgttcaaaccaggtccaagtaatgccaacatactgaatttagttgatatgtctctttaagtctcttttaatctgttaatggttgcccttccccttgtattttcatgctacctgttagttgaagaaatcaggtaatttgctctgtagaatttcacacattctggatctgtttggcttcttccttgtggtgccctttatagccagccctccatatgtgcagattcaaccaatctcaaatagaaaatactcaaaaaaaaacaataaaaataaaatacaataaaaataatgcaaattgaaaaatacagtataacaactatttacatagtatttacattgtgataggtataagtgatctaaagataatttaaagtatacaggaagatgtgagtaggtaatatgcaaatacatactatgccattttatacaagggacttgagcatcctcagattttaccatcagtggaggatcctggaaccaattccccatggataccaagggatgaccatatactgttcatctagtccctgtctgctttcagttcattattccagcaataaggctttgtagatggtggtgtggacttcctattgcattacgtcaggaagtgtgttgtctgatagacccatttttattaaggttaaaacagatcaaagggttcagaggtggccagtttgatagatccaccataaaaatctcgctataaaatatttcacctattagttgtagtacccattgaagatcatgttttctggacccattattccattaaggtctagaaaatggtgatttttctaatcctctaattccttctagatttattagacttcttcaaaaaagaaaaacccattcaaaaaacaaattttttttttgagacagggtctcactctgtcacccaggctggagtgcagtggcacgatctcagctcactgcaaactctgcctcttgggttcaagtgatcctcccacctcagcctgggactacaggtgtgtgccaccatgcctggctaaattttgtatttttagtacagacagggtttcaccatgttaaccaggttggtctcaaactcctggcctcaagtgatccacccaccttgtcctcccaaagtgctgggattacaggtgtgacccctgtgccaggccaaattcatttgaatttgatgaacttctggtgaccctgaaatttggttcacatgggaaaaggaaactaaatgacaatttttcctctgatttattgatttcaagaataatgagttgggctgggtgtggtggctcatacctgtaaccccagcacctttggaggccaaggagggaggatcacttgagcccagaagttcaagaccagcctgggcaacatagtgagaccctttctctaaaaaaaaaaaaaaaatttaggtggaagaatcacttgagcccaggaggaacagggtacagtgaactgtgcttgtaccactgcactccagcctgggggacaaagtgacaccctgtctcaaaaaaattatacattggtgctctagcatctttcataggttaccaaattatgcagccacaatcaagtaaactatcaaattattggtgggatcacatcaaaaactcaacttgaaacaactcctactggttgaagatatggcattttgagcatccaaaagtatactgacttatagaatgatgttttgtttctttcccacaggagttttatacacacacataaatatacacaacaatattaaattcctaggtggttaatttcttttaagccacatttttgatagtttctaattaattttaaactgtggtcagacaacagggattgtaagccttttgctttctggaattatgggaaaatcatttcctatttccctctaattcttcaacagctgtattactagtgacctcacattcatgaaattcatttttggcatgaaatttctaatgcagctcaagtgctgaagaacttcctacattcactacaatctaaattttacctagaataaattatgtttaataatttctgagaggtgacaggaggcatttctacatttattatgtctacagatcttccttttacgtgaattcactaatactaatgacaataataacaattacagataatatttacagaatacatgctatatgactgtgattcctccaagtattaactacttactccttgcaacaatcctattccacagtgtggcaggctgactctaaacaggccccccagtggtcctgtctccaggacttattcacactcttgtatcatcccgttctcttgagtgtggactatcctagtaacttacttctaccagtagaaggtgagggaatgttacttccatgattagattacacaagatggtaacttccatcttgctagcagactgtcctcccttttggcttgcatgccttgatgaagcaagcagccatgttgatgaggctattgtggccaggagctgcagtcagcgttcagccaacagccagctagaaactgagaatctcaatgcaacaggcctcacggaaatacattgggtaacaactatgttagtctggatgtggatccttccccagttgagccttcagatgagacctcagccctggctgaaatctgtagccttgcaagagaccctgaagcagaggacccaactaagtcatgcctatactcctgatccaaattataagatataattatatgttattttatgctactaagtctgtggtaatttattacgcagcaataaataactaatacatataagtactattattaccattttacaagtcagcaaaatgaggcacagaagcttagtatcttgtccaataaatcaaactggtaatcaagtggagaaagggagataatgacagataaggctaaagattttcctacattcattacattattctctcataggaatttgctgaagataaaccatgtttaaatggtgttggaaggcttttaaatcaacatattctttctctaatataaaatttattatgcttggaattgagcatgaaacacattttctcaaaaatgaattttctgatgttctgtaacatcatatacatttgaaggctttcttctattaaattccattatgaatcttctgatgctgagtaaggtgtgaatgctgtctaaaggccttcttacactccttacacttgtagggcttctcaccagtatgaattctctggtgttgagtaagaaatgaataaagtctaaaagccttaccacattccttacattcataaggtttctcaccagtgtgaatactctgatgttgggtaagttgtgagagcagtctaaaaggttttctacattccttacattcataaggtttctcaccagtgtgaatactttgatgctgagtaagttgtgagagcagtctaaaggcctttccacactcttcacattcatagggtctctcaccaatatgaatgctctggtgtgaaataagctgtgagtaactactaaaggtcttccaacattccatacattcatagggtttctcacgagtatgtattctctgatggcgaactagttgttgtcttaatctaaaagtcttcccacattccttacattcgtagggtttctcaccagtatgaatactctgatgaacagtaagttgttggcatattctaaaagcctttccacactccttacattcatagggtttctcaccaaaatgaattttctgatgtactctaaggtctggaccacatacgaaggctttcccacattccttacattcatagagcttttcagcagtatgaagtctctgatggcgtgtaaggtgtgtacactgtctaaaggtctttccacagtccttacattcatagggtttctcaccagtgtgaattctctgatgtcgagccagttgctgatgtactctaaaggcctttccacattccttacattcatagggtttttcacccgtatgaagtctctgatgttgagtaagttcttggagcactgtaaaggccttcccacactccttacattcatagggtttctcaccggtgtgaagtttgtgatgtcgaataagatgtgcacgctgtctaaaggcctgcccacattccttacacttataaggtttctcaccagtatgaattctcaggtgttgactaagtgttgagcgacgaataaaggtcttcctacactccttacactcatacaccttttctccattatgaacgatctgatactcagtaagaaaattgtgccttttgtaagtggtcattttttcagaggtaattttcacttgcccaaaatatccctcttgttgttccttttccccctcaatcttgcttttgcattcccaatcattcctaaaaatggaaccctgaaggctatagcttttaattctttccattatatcccactgaaatgaatatatttcataaatgtccttttctggagataaagtattggtcctgtatctggactccaaatctgcagtagtgatttctcaatgcctgctcagccctcactcaccagggcagtatcttcttgtcccttccctcacaaccatcccaggttc

SEQ ID NO: 14118 - RNA, 3545 nt, Homo sapiens
  source 1..3545: mol_type = other RNA
gctgggattacaggcatgagccaccgcacctggccattagctattctcaatcataagtcagagcaaggcagagtgaatggtaaatgagtgaatattgcaaaggaactcaaattccagataagaagtctgggaaaggtaattgttaagatcctttgacccttgataatttattcttgatttcatagaaaaacaatccaatgaaacatttactgcctgtcttcttaaatactcatttgtgtgtgtgtaccttgtcttaccattgtgctatttttccttctaacagtgttctcaaggatgtaccagttatacagtagagttaatttatttgtagtgaatagggatgcaaattcctacttctaattttcagttttaatcaccagaaaatgcatggctgcttgatggaaaatactagagtttaatatgaaaaccttcctgtcaacatttcagttttccctcattgcctcgtttccctaacaaagactccacattctccagtgtttagcagacaataaatcagtgctgtggctcatttaacactcatattggaagggatttattctctctaaagcttcagaagttgggccaaatactcaatttttatacattcaacccctcaaatccaaaagatgtgatatgaaccaaactaacacaaacaaactctctgggggaaaaataatactgtggatttaaaatcactaatagataaaatgaggacacattcctctgggtggtatagaatttctctcctctgctccagagggtgcattgcttttcagcagcataaatctatctcctttggtcaaagagatgatttagtctccagagccaagacaaaaatcctgttggatattagaatttggagagttccatggcctccaaacaggaatttatataccagagctggtaatggtccatctagtcgagcctcctgcttcctcctgcatcgaatgatggatgtgttagaagacaggaataaactcaccgtgatgcccctaattgagaaaaaaagccacaccaaggaaatttcgtcttaactctggtactgggttattttattccatcatgcctgagacctgatagctatttacctctatactactgttacagagaaattcttttattttatttttatttttggtaggaacacactattaaatttctcataagcatttaattcttaattgaatcttattaacttctgctgattaacaactcactgtagagtgaacaagcaatcacattccacctcttaattttgcttaaaaacttccagctaaatgtacataaaatagtgatacctcttactttatttcttaatattatatgtctataaaaaatgtgacccactggaagtcaacacataaaaaattctctgtaattagttataaaatgtattatttagttattaaactacaaggagtgaaagttcaattcatgacttgtgagtgtttcaagcctactctgtattatttgcttaaaccttttaagaacctcatatttctttactaggagaaaattgccactgagctagactacattaacatgaaatgtgtttaacaatatccttgcttggaaactactaacaatgtgttaacagttttccaggacactgtggacagtgcattttattttttttgacaacaggactgcaaaccactttattcaactctgtattacgttgttaagcctccgatggaaggactttaagtaaacagtctatgtcatcaaaggactcaactcactgtcatcacctatagaatgttgagcaataagggcaaggtcaaatcttgcattagaagtctgtgctactgtgggttcactgctactcaggctttgagagcaggcatttatgcttgttggcagactaattaagggaaatgatatgccaaaagagttctcgcctcatcattttttaaaatgtgtttactcataactgtgcttggattggtggtcagaagggctagaagaagcactaatcctccaacaattctctaattctttttgcacgaacagcttacattatcacctgttttgagtgaaaagccataaattggtcccaggtaattgtaaatcatatagtcaaatatgaaagctcgttcctctgaatgataataggttaacaatcaaatatttatttatatgattaatgtgactaaaatggggtttatttaaagagcatagaatgaacatcaagagaacaggacttctgcctgcatgccccagatttgaatccttggcccaaacagtcatttctatgtgcaattaggcaagccatgtattgtctattaacctacttcatgagagtgcgatgcgaagattataacttttaacatacttttagatcattgtttatattattaccactatcgtcatattttatgatttataaattatgtgattaatgtgaatacataaattatgtgaacagagtattctacgactaaactacttttaaaaaccaaagcagattatgatttgtttgaaagatagagaaaaagaaataaaactttgacaataatatgttgctcttatatagcatattccattgttttccttatttgagtctcacaaacatcatgtagggtatgttaattattattataaaactttgagaagagtgtatttttccctctaggaactaagctcctttagaaaaaataatgtgaatgtacttttgtactgttacaaggtagtactagactgataaatatgtcctcacaaatggacgtagcacttgaaaggttttggagctatatggctctgtacatgtcattattatattgtttttaagtgaatatcattttctccaagcccatgcatatgtgtataagcttctgttagaggtaaacaggtagatgacaagttgtttctttgcttaaattttagttgcaaggcaaatttcctaacagcctctgttccatgtacctcaggaacttggtgtcagaaaccttcaggcagtagtcagtcttgtctgtttctagagatctgttttggagttgattcatggattggtatatggtaaagataaagcacttggttccaatccctggagattctggagatttagagaagtgggattgctgaatcatatggtagttctattttagaattttccttggttttaggaaaacacatggcaccttttaggaagtttgcggaaggaaacttcttgtttttcttcctgaccagaaaaaaaaaaaaaaagccaaaatgacatttacttattaaaaatgatcagtttggaagtgtgaaggactggatttcaaaacagtactttccaatctggatgaaagataatattcatatatgatcaatacaatctattcaaatccaatcagcatgatttttatattttccctttttcttcttctagaaaaatcacattaatattttgattaaatcaaccacatagaaaccccgagcttcaaaatgaagtgaatttccaccaatttctttgtgcagctaggaaattttggaggttcctcttgttttcccacactagagggagagggcatgagtgagactaggctgatctccacgcagag

SEQ ID NO: 14119 - RNA, 3151 nt, Homo sapiens
  source 1..3151: mol_type = other RNA
gctgggattacaggcatgagccaccgcacctggcccaaagcttgattttctaatttctagggttcacactacttctattattacaaaaatctcaaattctatgcacctagtggctagaatgaataattaaggcctctaggaacttggaagaaggacagattggagttgtctggaaaattttttatggaggacacaggatctgacccgggagttgaagactgggtaggacgttcattaatggagaacaggagggaagtctcttggaaggattaatgcgagcaaaggcacaagggtgtgcacaaggatgtttcatcgagtagagtataaaggatttgtgggaaataagacaggattagtaaattggggccaggcaatggagtgccttaaagaataggataagtagttcaagtttaatccttcctgtaagcaagtttcctttaaaatatgtttgagagtgataaaatcaaattagacttacagagtaaacacatatgagcgtgtgtgtgtgtgtgtgtatttagccaaaaccaaaagcttgtcaataactatattatgtaaaacttcttttctataaaaacagcatgctgtctcccattgtccctctatatatgaaaacttgctgccaggaagttttcatatatgcagggtttactttcccattacttttcctagtgacacttagttttcaccatgttctgtggcttacgtgttctgcccctcacaggtacccctatagaaagaatactccaaaacaccaagggagtcaccaagagagaaagccaggcagggtgggaaactgaaaatctccactgattctgcagagaagctctaaggaacaatccttccatttcaaagcatcagaagggccaggagctcaattcatccttcacatttccataggatgaaacattatttgttccctttaagatactatgtgatgaattaccgcagaagagatggaaggagaaaaaaatgggaatacaatagttaacacttctgttatatttattatttaccagaagaaaacaataataaagcaaatgtttaaaaaattttctttaacttctgcttcgggaaatatgactctaaatttcacctgagtcactcaaattgattgcaagtagaaaatattgcctctaaatattatattttatctccttccaccttcctcttcagcccctacttcttcatggcccaaacattctgccttttacaaatacccttatcagatggtagcattgtttccagttctgccacgtggatcctaaagtattgctgctgacatagtctccatgctgtaatccaagagtcactatttccatttcttgttcttctagatggctctgttgcctcttacgccagttcttttggcagttgcacaggtttaagataggcgacactgctgtgacgaatgtcgtttagcagctgatctctgggagtgatttccaccaatgggggtggcctgtttctcggcactggcttgagcgttttgatgacatctttgaggttggttttctcgggtggttctctggcttccggcatccgagatttgcgctggattctcttcagcttcaccacccggaaggagtcagggtctgtcctgtacttcggggcctgcgatggctttttcatcatttcactgcgttgactaaaggggacattttgggggttgggaggccgaggtggcggtggctggaagaattcctgcattctggaatctggcttgggtcctcccaacagctcccacatcccagggggcagccccaacccattctctaacatggctatcagcttcttctgttccttgagttgctgctgtttttgctcttcctgtcgtttctgcctttgtttatcctgattcctggtgagcagattagtgaccaccattctgggacccggaagctcaaaatggtagcccatcttcaggagagtgttgtttgccttcaaaagcctggctatttccatttcagcatggtgacccaacatgtgcctctgattgtgaaaccgaagctcagttagcgtctcattaaactggagacacctcatgatggccacaatccctttacctgtgatgaaattggactcgatgttgagagtggtgatgcttctattttcacgcaacatgttagccaaggcaaatgctacattctcatctgcacccacattggctaaactgaatgttttgatgtgcttgtttttcttcattgcattgacaaagtccagtaacatttctttggggatgttttcaatgttgttcaggttgagttccttcatgtcaggatcatttttcctaactctcctcaagctcccatccaggtctgtctggtttcctgaaggccttgtacttaccttcaaaaagctggtgtctagagctaacttcttaggatctaatttcgatatttttttctcactttgttcttgggcctctggtctgtctctctgttctttgaatgctttgtcagttacctgctggcagttgttctcacaatttctaatttgttcctttgctttgccttcctcttctctgttcgtttcttcactctcttcaccatcatcttctccttcgtcgtcatcatcatcatcttcttcttcttcatcttcttcatctgtttcttggatattgctgctgccctttgattctcttttatttgcaactatttcattattgagcttttcttttaaatactgggccatatttttattacgtttttctatttcttcatgctcttcttgagtcttttcctcggatttcacaaaggtgacaggaactcgttcctcttccagcatgcgcctggatgccttttcccaatacatataatcaacaagagatttatgattgaagtttcctgtcggtggcttgtcagtttgatctttctgaatcattcccacgggaaggctggggtcaggggccatgacttccatttccgactgcagttctttcagttcttcagcagacaagttggccaagatttcatcttcattaatctcctcatcgagaagttcttcttgatctgaatttctgctgtgctctgacattattttttctaaatattattttaccttgagatatttttttttttttcccaggaacctcagtggtttgctgagcagctaggagtgatcacagctaagctcttgccggatctatatt

SEQ ID NO: 14120 - RNA, 3245 nt, Homo sapiens
  source 1..3245: mol_type = other RNA
gctgggattacaggcatgagccaccgcacctggcccaaagcttgattttctaatttctagggttcacactacttctattattacaaaaatctcaaattctatgcacctagtggctagaatgaataattaaggcctctaggaacttggaagaaggacagattggagttgtctggaaaattttttatggaggacacaggatctgacccgggagttgaagactgggtaggacgttcattaatggagaacaggagggaagtctcttggaaggattaatgcgagcaaaggcacaagggtgtgcacaaggatgtttcatcgagtagagtataaaggatttgtgggaaataagacaggattagtaaattggggccaggcaatggagtgccttaaagaataggataagtagttcaagtttaatccttcctgtaagcaagtttcctttaaaatatgtttgagagtgataaaatcaaattagacttacagagtaaacacatatgagcgtgtgtgtgtgtgtgtgtatttagccaaaaccaaaagcttgtcaataactatattatgtaaaacttcttttctataaaaacagcatgctgtctcccattgtccctctatatatgaaaacttgctgccaggaagttttcatatatgcagggtttactttcccattacttttcctagtgacacttagttttcaccatgttctgtggcttacgtgttctgcccctcacaggtacccctatagaaagaatactccaaaacaccaagggagtcaccaagagagaaagccaggcagggtgggaaactgaaaatctccactgattctgcagagaagctctaaggaacaatccttccatttcaaagcatcagaagggccaggagctcaattcatccttcacatttccataggatgaaacattatttgttccctttaagatactatgtgatgaattaccgcagaagagatggaaggagaaaaaaatgggaatacaatagttaacacttctgttatatttattatttaccagaagaaaacaataataaagcaaatgtttaaaaaattttctttaacttctgcttcgggaaatatgactctaaatttcacctgagtcactcaaattgattgcaagtagaaaatattgcctctaaatattatattttatctccttccaccttcctcttcagcccctacttcttcatggcccaaacattctgccttttacaaatacccttatcagatggtagcattgtttccagttctgccacgtggatcctaaagtattgctgctgacatagtctccatgctgtaatccaagagtcactatttccatttcttgttcttctagatggctctgttgcctcttacgccagttcttttggcagttgcacaggtttaagataggcgacactgctgtgacgaatgtcgtttagcagctgatctctgggagtgatttccaccaatgggggtggcctgtttctcggcactggcttgagcgttttgatgacatctttgaggttggttttctcgggtggttctctggcttccggcatccgagatttgcgctggattctcttcagcttcaccacccggaaggagtcagggtctgtcctgtacttcggggcctgcgatggctttttcatcatttcactgcgttgactaaaggggacattttgggggttgggaggccgaggtggcggtggctggaagaattcctgcattctggaatctggcttgggtcctcccaacagctcccacatcccagggggcagccccaacccattctctaacatggctatcagcttcttctgttccttgagttgctgctgtttttgctcttcctgtcgtttctgcctttgtttatcctgattcctggtgagcagattagtgaccaccattctgggacccggaagctcaaaatggtagcccatcttcaggagagtgttgtttgccttcaaaagcctggctatttccatttcagcatggtgacccaacatgtgcctctgattgtgaaaccgaagctcagttagcgtctcattaaactggagacacctcatgatggccacaatccctttacctgtgatgaaattggactcgatgttgagagtggtgatgcttctattttcacgcaacatgttagccaaggcaaatgctacattctcatctgcacccacattggctaaactgaatgttttgatgtgcttgtttttcttcattgcattgacaaagtccagtaacatttctttggggatgttttcaatgttgttcaggttgagttccttcatgtcaggatcatttttcctaactctcctcaagctcccatccaggtctgtctggtttcctgaaggccttgtacttaccttcaaaaagctggtgtctagagctaacttcttaggatctaatttcgatatttttttctcactttgttcttgggcctctggtctgtctctctgttctttgaatgctttgtcagttacctgctggcagttgttctcacaatttctaatttgttcctttgctttgccttcctcttctctgttcgtttcttcactctcttcaccatcatcttctccttcgtcgtcatcatcatcatcttcttcttcttcatcttcttcatctgtttcttggatattgctgctgccctttgattctcttttatttgcaactatttcattattgagcttttcttttaaatactgggccatatttttattacgtttttctatttcttcatgctcttcttgagtcttttcctcggatttcacaaaggtgacaggaactcgttcctcttccagcatgcgcctggatgccttttcccaatacatataatcaacaagagatttatgattgaagtttcctgtcggtggcttgtcagtttgatctttctgaatcattcccacgggaaggctggggtcaggggccatgacttccatttccgactgcagttctttcagttcttcagcagacaagttggccaagatttcatcttcattaatctcctcatcgagaagttcttcttgatctgaatttctgctgtgctctgacattattttttctaaatattattttactagaaaagaagaataatcaaagatgatttttaaaaagaaggaaaaaagcctcaagaaggtcccccagttaacgagtgtcccaagttaacacacccttgagatatttttttttttttcccaggaacctcagtggtttgctgagcagctaggagtgatcacagctaagctcttgccggatctatatt

SEQ ID NO: 14121 - RNA, 2250 nt, Homo sapiens
  source 1..2250: mol_type = other RNA
gctgggattacaggcatgagccaccgcacctggcccacattgttatacagtattctatttgaaccatgttaaaatatcatcatttgtaaatccacagaggagcctggtgaattcctaacacatattttctgtcttgttaagctgttgaattgcatcatggtggagaaatgtgtaaatagaagtaatgatcttggtgtttgtaaaaggggtatttgaaaggttcccgaaagtgtgagggggctgatagcagatctgcagcttctccccccgtgcactaaagccaatcataattctttctacctggtttgtgtcatcctccattaggagaccccatcttcagaaccaatggaggaagaggaagatgacgacttggagctgtttggtggctatgatagtttccggagttataacagcagtgtgggcagtgagagcagctcctatctggaggagtcaagtgaagcagaaaatgaggatcgggaagcaggggaactgccgacctccccgctgcatttgctcagccctgggactcctcgctccttggatggcagtggttctgagccaggtgccttcagagtgtcccctgttcccccagtcgtcctcatggatttccattagcccctctgttgacatctgtagccaagggaggccaagcagcagcacttcattcaggtagattcaggatatacacaccagtacctcccattcctcctcttattccattagcctttgtgggggcaggggctcacctggttaatgcagtgccccaggttttgaagggcccatcactttgtttgctttgaggtggtcatatcgggtgagtcatgtgctaagttctcttcccagctgtctgtgagatgtgtggtatcgtgggtacaagggaagccttcttctccaagaccaagaggttctgcagcgtctcctgctccaggagctactcctccaactccaagaaagccagtatcttggctaggttacaggtgagaggcaatcacttggatccttcccggtgcctttggtgctgagacaggaaccaccaagtgactgaaggccagggccaggaaagtttgaaaaggtccttgcttgtggccagctggtatttattatgttctcaaacttcagaggacagtagaatccatttgtggagctttttaaattataggttcctgaagctacgctccattacctaccatcatcccccagagtctggtgtattcagtacattttaaacaagaactatgggggagtctgacacccttggtcttcaccccacacttttataaatcctttcaaaggaagttgggaaacaggcccaaggttcaccagccacggtggcttcaggaagaccatgcctcctcggactccatgtcacaggcagctacctagaaagtcttgccaattttctaaattactgatatttatagaatctttagagatggaaagattcttggatgtggtgttgaacccacacatttattgataagtatactgaggtccaaggaggtagaatgacatacctagtgtggctctgtaggaggagaatggcggaattgaggctggaacctcatctcaggggcctcatcttaccttgtttcccagtagctgggaccagcatctgcaacactgcttcccaaatttgcctgcatgttgggatcacctctgcaggtcccacagggcccttggggtccaggctcctggagtggctgctgcgcaggctcctagtctgactcgtcctctctgctctgcagctctggtcttgggcttcgactgggggaagttcctgaaggatcacagttacaaggctgctcccgtcagctgtttcaagcacgtgagtgccctggagctgagggagggaggccggggagccgggcctggagctgctcctccacctgcttcaccagggcggcttcaggctggacagtgacagtggggaggtctgggcaggagacggatggcgttaccactcgctccatttcatgtttatgtcaaaaaaatcctcctacaaacacttctatcacctgcttggcttcactcccggtctgaagcccttcagtttatttacatgatggaacttggtgctagctgatgtcgaagggtctttgcagtctgaaacccttctctcctttctcccccatttgcagcattttcccatggaaagcagggtgcttctgtagctggcctgggccccgtgggccccgagaggcagatgtggatgctcctggagccacttctgtaaaaggctcctcgatgcgg

SEQ ID NO: 14122 - RNA, 1349 nt, Homo sapiens
  source 1..1349: mol_type = other RNA
gctgggattacaggcatgagccaccgcacctggccctgttcaatccatttatatgagtgaggaactcctacaacttactgtaatctctcaaagtacatcctatattctcacttagagcaacagagcagaaatacaaacatcaaggattgtaacatcaatttattccagggtagatcggcaaacttaaaagtgtgatgtttgtcttctgtcttccacacagctctatcactgcttgtagtgcttcaattcataccaactatacttataggcactatttgggtctattttccacagcatcttctgtgacttaactatataatgtttggaaagaggatttccctgaccgtctatgatactagctttgtaaatcctattaaagaccatcaattaaccataactcaataatccaaacactattgaagtgataactactcatctttctcatgcttttccagtctttgttagtcttcaaaacagacaaaatgtttttgcatataagatgttaatttggggcataattgttttaaggagtgtaatagctggtgttctgacttggttagaaattcaaacagctcttttagatacctgatgaagttttgttagttaatcaaaggctttattatatcaatgccacatttaatctcttttgcaaatttctaatcatgtgcaagaatttctattttatttaaccatggctgtttttgtgggggaacatgctggcaatgtgctgttgagaatttcattttccatagatatctgttaccagtataacaaaattgacagcatctgctgatgaaatgcactactcaaaaaaatttttttaagatttgtacttttctccaatatttttctgaagtacagctctttacatcttttccagggtctgatggaaggctttctcatttcacagctgacagcacatcattttcacctttacctctattctcatcatttgttcatcttgggaatagtttcttgtctgccttttgggaactagattattgacttttcatgttccagggagtctgcaactctgaccccagtttcagtcaaagaaattgttgtccaaagtccttcgcgagggtccgtggcttcattcttgaagtcagtgagaccaagaatccaccaattctggagacattattattatggtttcaagaattgcttcaagtaacttcatttagagattgatgatgaggacacaactgcagtcatctgaaatacttatagaatgggagttagatgaatttaactccttggtctcttccaactctaaaaattatatgcatctatgagttactagcctttcacacatttggttcagcagtaccatctgcttctgcatttct

SEQ ID NO: 14123 - RNA, 307 nt, Homo sapiens
  source 1..307: mol_type = other RNA
gctgggattacaggcatgagccaccgcacctggccgtcttgctatttcttgattcctcaattttagaccttgtgctgtgtatcatccaggtaccctggccccattctgcatcttgttgcctgccctggcgctgatcagtatggacattttcaatgggcttctttatcctctgactcctgcttgagtttggccaagagaatacctgttttgcagcaataacaatgattgtgattgtagcttcaatataaattcgttggtttgtagacagtaccacacacactgtatcttctcggcctaaaaattcgag

SEQ ID NO: 14124 - RNA, 2857 nt, Homo sapiens
  source 1..2857: mol_type = other RNA
gctgggattacaggcatgagccaccgcacctggcctaggatggattttaaagatgggcccgaacatgcagggtttgacatgaggatgtcgagaggccattccttagtaggcagtagcagacctgtgctccatcgccagaattccgttgtctcaggaatgttcaatagatggaatcctgtgtggcctgagatgagtgtctttcatgccgcgtgacacccttgaggcccgtgcaactgttggtatgtcaacagttagctgcttctcattgctgagtggcgattggtcctgtcatggtttattcagccatgtggtggatggctacttgtcttctaagccacttgccttctgatcgctggactgactctctcgccctctcttggtgcagtcctcaggaggctcggtcacactctccaagagcacagccatcatctcccacggtaccacaggcctggtcacatgggatgccgccctctaccttgcagaatgggccatcgagaacccggcagccttgattaacaggtgacctcggggcacagggcagggcaccgaggcaggcttaccctggtgcagtcgaaaacacggtcccctttcctcccgccaggactgtcctagagcttggcagtggtgccggcctcacaggccttgccatctgcaagatgtgccgcccccgggcatacatcttcagcgaccctcacagccgggtcctcgagcagctccgagggaatgtccttctcaatggcctctcattagaggcagacatcactggcaacttagacagccccagggtgacagtggcccagctggactgggacgtagcaatggtccatcagctctctgccttccagccagatgttgtcattgcagcaggtaatgcccagccccgggcatcctgtgcaggcggtgtccttgcagctctacccagctcttggctctgggaaaagggaacaatggacactgtcgggcatggacgtgatggggcttccagaagagttactctgggcctccagggtgacatcaaaggacaggggtgcctcttaaggtgaccttcaagccacagccctgttgttggagacaggcatactcccgttacagtcgtcaccacatggctctgtcccagagccatgccctgtgtccttcagagaccgcaggaggaaaacaaccacttctggtacgaggtcagggcccttgagagaaggtgctgtttggctgggccaccaaaaacccctcacccctgtgagcacactcagtcccctctctggtggaacagagctctgcctgtagtcctgggtcccagccctgaaacccacaggtccagcggtggccagggacacaggcccacccctgcaagccagcagaccaatcggcagacacctgaaacacgaagttcacggcagggtcaggctttctgtcattgaaagccctctagacaggccgagaaccagagctggttttttaaggacaccagtgagtctggagatttttttcttttgcttcggtcttttgcagctttctctaataagggttctcctttttcacccaaataattgcctttccatctaatggcccaaatggtcaaatggcatctaatagtctcatatgaccgctgcctctctggcctcgccctgctgctgaggtcagcatgaaatggaactttccacttgtccctttcagtaacctgaaactttcactgtagacgtgctgtattgcccagaagccatcgtgtcgctggtcggggtcctgcagaggctggctgcctggagtcgcaagacgagctgaaaaaggagccaggcactgaaggacaaagcggtgttgactttgttcatctgtgtttcccagtgcggtccaattgacggtggtttccaagcgcctcatgtaactgattaggttagggtacgttccacgtcaggtgaccagaggcagtataaaaggcagcctggaaagcagaggtccctctccgccccttcctccatcttcctggatgctgcatcgcttccaggggggctgctccagcacctgttctgggactctgctccacttgccaacatttgagtggattcatttgtgttgtagtcaagattcccgttgtggcacaaggacacatgcactcgtgtccaactccaaatagtagcttcacatagtatgtcagcactctcccaccatcatctcttctagaaggtcttccgctggattggaaatggcctgctgcaggacactcagcagctttcagtagttcatccagacatccagttggaagtgggatttccagtatttccactctgcttggaagacttagaaaatcctgaggctgctcagagggtcagcttcccatcgctgtgtttcagtaaaacttcagtcttccctggacaagtgaggagacagaaaatgtctagtctctggcacatcttttgcaagcaatggcggctcccaggaatcaatactatcaacgaatatatttttgagattctggtcaaaagaagagtcatcctgcaatttcaggtaggatggagtggttctgtggctcctgaggtgattttgaaaagatcttgactctcagaaggaccaaggaggacatttctggcatttccagaccaggaagagtgactgatggacctccagtgttacttggaaaaattttgttggacagctttgtaacaagaggatcttgctttggctttcaggccttcacataggttgtttagatcatggaagtgtttctgcatttctgcataggctcaggatgccttctcaagtcgtccctggaggaggaggaggtgaacctggagctcccgccggcctctgggcgctccttggtggaaggagagggacttggtcctgagcctgccccggatccacctac

SEQ ID NO: 14125 - RNA, 1898 nt, Homo sapiens
  source 1..1898: mol_type = other RNA
gctgggattacaggcatgagccaccgcacctggcctggtttagctttaaaaaaaaaaatctttcttgtgcttactgccgtgtccccactgcctggtgtgcggtgacattgggtgatggcggggcgttggaccacaggactggtgtgtgaggtgccgcctagagatggggtgacctggtgatctgggagtgatctggggagcccaggctggagacggggagggtagctactgcagctcctgccctggtgccgcacttctgtcccgggaggtggcgctggcccagactgtcccatcccatgcctcagggccccctcctgctgcactgggccagccgtgcttgccagtcccagcgggttctcggccccgcgacagcctccttgctcagagctcttgggcgatgcggctgggttggacagagcagatgctggccatgcctccactggggacatgcacagggcctggggtctgtggggacgtgaggaacggtctgacgatgacgacacacccagcatcagcccgcctccacctggaggcccaccagcacctggcccgggacccaccctctctccagaacctgtcgctgtgccccggacggtaggaccggtgatgggtctgaaaggcagctccatccactcctggccgtgcgactttggggacctggcttcctgcctaagccccggtttccctctctatagaatgggctgacagctgtgcccgaggtccagggcacaacggagaggggagtgctcacatggcgagcacacggtgagaggagaccaggctcgcgggagctgctgctatttgttatttccaggggactgggagcctggagagtgggcagctctgctgatggggattaggagaagcagagagatttacactcatcttacagagtcagcggtcccgccacccacagcctcgcagccctcgaacctcggaggcccccacgcccaattaacagacaggagactgaggccccaggaggggaggaggtccccgcacctggcctgagaatacttgggtcacctcctgcctgacactgggggccagtccgctgccagcaggacgggtggcgatggggtgggagacgggatgggggcagggaacccagcagcctgtctctctggtcccgctccccagtggtggtggcctggcctgaccacggttgctccatgacctcggcctaggccaaggcgtggtggctgtcaccagggcacgtccccggttctcgggttgggccgaggagggggcccgggagggcggcaggctcaggctggcggccaggccctgtccagagcctgtgcatgttccttggccagcagccgcagggacgcctcctccagggcgaagccatctgcgaaggtgggagcaaaggcatgaggcccgaaggacgcttgcagccccgggcccgggcccaggaggcgggggaggcctggcacggccggcggtccggggcccaaccagggctccaggggcagcgacatggccggggggcgggcgaacggcagcgctggggcctcggggagtctcggagctgccacggcacccgagcctgactccagccgctcctggcggcgccacttggcccggcggttctggaaccacacctgcacgcgcacctcaggtaggtgcaccttggctgccagctcctcacggctgtacacatccgggtagtgagaggcctcgaacgcccgctccagctggtgcagctggtaggtggtgaaggtggtgcggttcctccggtgcttcttcttgggggcctcctcgcccggccccagacccccaccctcggttgccggcccctcgcccgggctcaggaacatggctcccaccgcccacggcagcccctccgtcgatttccacgggacacctgccccagcgggcctggcgctgcgtct

SEQ ID NO: 14126 - RNA, 2157 nt, Homo sapiens
  source 1..2157: mol_type = other RNA
gctgggattacaggcatgagccaccgcacctggcctggtttagctttaaaaaaaaaaatctttcttgtgcttactgccgtgtccccactgcctggtgtgcggtgacattgggtgatggcggggcgttggaccacaggactggtgtgtgaggtgccgcctagagatggggtgacctggtgatctgggagtgatctggggagcccaggctggagacggggagggtagctactgcagctcctgccctggtgccgcacttctgtcccgggaggtggcgctggcccagactgtcccatcccatgcctcagggccccctcctgctgcactgggccagccgtgcttgccagtcccagcgggttctcggccccgcgacagcctccttgctcagagctcttgggcgatgcggctgggttggacagagcagatgctggccatgcctccactggggacatgcacagggcctggggtctgtggggacgtgaggaacggtctgacgatgacgacacacccagcatcagcccgcctccacctggaggcccaccagcacctggcccgggacccaccctctctccagaacctgtcgctgtgccccggacggtaggaccggtgatgggtctgaaaggcagctccatccactcctggccgtgcgactttggggacctggcttcctgcctaagccccggtttccctctctatagaatgggctgacagctgtgcccgaggtccagggcacaacggagaggggagtgctcacatggcgagcacacggtgagaggagaccaggctcgcgggagctgctgctatttgttatttccaggggactgggagcctggagagtgggcagctctgctgatggggattaggagaagcagagagatttacactcatcttacagagtcagcggtcccgccacccacagcctcgcagccctcgaacctcggaggcccccacgcccaattaacagacaggagactgaggccccaggaggggaggaggtccccgcacctggcctgagaatacttgggtcacctcctgcctgacactgggggccagtccgctgccagcaggacgggtggcgatggggtgggagacgggatgggggcagggaacccagcagcctgtctctctggtcccgctccccagtggtggtggcctggcctgaccacggttgctccatgacctcggcctaggccaaggcgtggtggctgtcaccagggcacgtccccggttctcgggttgggccgaggagggggcccgggagggcggcaggctcaggctggcggccaggccctgtccagagcctgtgcatgttccttggccagcagccgcagggacgcctcctccagggcgaagccatctgcgaaggtgggagcaaaggcatgaggcccgaaggacgcttgcagccccgggcccgggcccaggaggcgggggaggcctggcacggccggcggtccggggcccaaccagggctccaggggcagcgacatggccggggggcgggcgaacggcagcgctggggcctcggggagtctcggagctgccacggcacccgagcctgactccagccgctcctggcggcgccacttggcccggcggttctggaaccacacctgcacgcgcacctcaggtaggtgcaccttggctgccagctcctcacggctgtacacatccgggtagtgagaggcctcgaacgcccgctccagctggtgcagctggtaggtggtgaaggtggtgcggttcctccggtgcttcttcttgggggcctcctcgcccggccccagacccccaccctcggttgccggcccctcgcccgggctcaggaacatggctcccacctggtgggacggcagcgggacagatggtggggagacggctgggggggctaccggcagggacagggcaggggagccccaggcttgcctcccggctccggggaaatcggttccctccactggggccggcatgcgctctgcatccccaggctgtcctcctcgggcttgggggggtctcctgctgtgcctctgtctgctcttccttctctctgtgtgtgtcaccgtccctgttttctcttcccctctctgtgactgtcacggccgcccacggcagcccctccgtcgatttccacgggacacctgccccagcgggcctggcgctgcgtct

SEQ ID NO: 14127 - RNA, 15862 nt, Homo sapiens
  source 1..15862: mol_type = other RNA
gctgggattacaggcatgagccaccgcacctggccttccctgcttcctctctagaatccaattagggatgtttgttactactcatattgattaaaacagttaacaaacttttttctttttaaaatgtgagatcagtgaactctggttttaagataatctgaaacaaggtccttgggagtaataaaattggtcacattctgtaaagcacattctgtttaggaatcaacttatctcaaattgtaactcggggcctaactatatgagatggctgaaaaaataccacatcgtctgttttcactaggtgatgccaaaatattttgctttatgtatattacagttctttttaaaacactggaagactcatgttaaactctaattgtgaaggcagaatctctgctaatttttcagattaaaattctctttgaaaaaatacagtctgtattcatgaattgtaaaatatgtgcttcagtgagcagagttagggaatccaggaacttgggtggggaaaaattacatctttatttgcactaataatttctaactgcaatttagtatttatttcaattatgaatttgggcagcattttattagcagtatccatgattttgtcaatagaaatctcagatattttcatattacagatgttacagatttcttgaagtatctagttacgaccccgagataaggctagtctaatgtttagtgaatagttttagacttcttaacagatttcatttttaatcacagactaattaattattgagatgcataaacaagtgtgattgcagaggcctactatcataaggaggcgtggtggtcaaacaatggcactgaactcagcttgatcagatcatttgtccatctgtttttttctccactgtctcttagagcagaatagccttgaatggcaagccatgctagctgaaaaaggtttttacccacaacctgccccttcaactaactgctttagagtacgtttgctatttttagaattcctcttattggaacccagcttctaatgtggaaaatttaagtatagttggctccttttatttgtgggttctgtatcctctgattcaaccaactgcaggttcaaaatactaaaaataaaaccccacaataaaaaaatacagtattagcaactatttacataatgttcacattgtattaggtatcaaataatctggagatgatttgaagtacacaggaggatgtatgtagactatctgcaaatagcacattgttttataagagacttaagcattcgcggactgtaatatccaagggggatcctggaactaatcccccacacatgccgagggatgactgaaattagaaatgttcaagcatgtacaactttctaccatgcctgtttgtgttggtataaatcatggaacatcaaataataagacaaaatcctccaggtgtaagcatcaaatactagtcctcttgctgttttagtgagttgccatgttattgaggaggactccagatgagaaataacattgcgatctgtattatctctgtgagagcctcccagtctgaatttggcttggacaacagggatactgtttaattcggctgcaatgtgattaagatcttttgagttaatgatttcttcatctttttagtgggccatggatttgtgagaacacatctttggaaacaagtaacactaactgtaatatagtaaatactgattaatcatgaaataccaatatagcttttaaaaaacactatgtagatgtaaagttgatacaaagacacatggaaaactttcaacagtattaactctaagattaggacaactttctctgaatctctcactcctacatatttgacataagtaatgagatgctatgtaccaagaactatggctcagttaaaaatgaagaaggttcaaatacagtgtggtgaaaatggtgaagtcatttttatttcagtacttgacaaaataccccataaaattcaaaacttctaccattatacaaaaataggtctctacaagtgatattatctgtcttcatcaccagtagaatatattaggcaaaacatgtaacttcagtagccttataagaaaagtgcaggacacctcgagctacacattcagcagtattgtaatgcgtaaaagtttaatcttttcacccatttgataaatacacaaggtttataatttaatgttttaaattagcattccacaaatatacaggtaattcaataattattgtgcatgaatacatacacaatgcttatatatacaaattccagtttgttttcatgtgctggcaagggatttgtatacaatcataagctgtgttcatattggtcccattgaatattcacaatacaaaagcacaaaagaaccattgatttacaaaaggaaatctatttaaaatcacttcaattaatgatgtttcaaaggattatcttctcatgccagcatgaaattgagtagttgaacctatgagagaaaaacaggaaattcaactgatttcaaattacattgctacctgtatcagacccaccagagttcacacaaaggaaattattattattctccatttttttaaagccctttttttccttaaaatgtcctcttcatacttaaactgagtctctccccactacccccaaggtggagtgttactctgttgcccaggctggaattcagtggtgtgatcttggctcactgcaacccccgcctcctgggttcaagtgattctcctgcctcagcctcctgagtagctgggactatccacacatgccaccatgtccagcaaatttttgtatttttagtggagacggggtttcaccatgttggccaggctagtctcgaactggttggtcttgaactcctgacctagtgatccgcctgcctcggccgcccaaagtgctgggattacaggcatgagccaccgcgcccagcccatatacttaagctgacttttaagagattttgaatatatatgtaaaaatcaccatgactggctctatggcaaggtaggtgagactaatatttagagtttttttaaagtgctctcaaagttggatgttctatacctcatacatttttgaaaaatcttttggtcttcaaaatctgggtcttgtgaaatttggatgctcaaaacaaaacaagcctaggcaaaccaacaaactcagctatgataataaaagtttcctattactacaagatgcttgggtgtaaacaaatgatttcttgaaggaagagataaactactcaatgattcaaagtctctgaatcaggagtgaactgaagtgagatagggaaaagaggttttccttccatgaacagggaatccacctttattttaaagtatgacttgttttttgtttttgaacaaagaaaaaataatccttacaaagtattttaaatgggatagtttttttcgatgatacataaaagcacaatatagtagcagggataatggttacattaagtgcttaaagtaagtgcttcctccttaactccacccgatttgcatgccttaccactttcttttttttttttttttctttgagacagggtctcgctctgctgcccaggctggagtgctgcggcacggccttaccactttctgccatgcgctacttaggaatacgttctccagttaggctctgtagactcagagtaccttgcacactggtgctcattgtgcattttgtgtcatcagtccgctgaatgaacatagtaggaaatcatttttgggaggagtgggatctggggtgataaatcatattttcacttaaattatttaaagtcagtttctctgctggttacaagagtttaagctttggctaacttaataattagctcatgcactaaactggaagctttgattatcctaatgagtgtgaaagaatttcaaagaaaggggagctgtgggtctcgcactgtggtgctgccaagatgtggttaaactcagagcacctgactgtatagttccaagtcgtctttgcagtgcctctagccgagtgatataatctgttagggctctgtcaggatcgtaattctgaagctgagaacatgctaaagaaccaggattgaaatcagctggagtgcctgggtacctattctgaaatggtaaaggggacctaatatagtccagatctgatcttgagcgatacgtagtatgtcttggttctccatataactccagcccaccagaagaatgataaaatgagtcagtcttttctgcaccttgattcagtccaaagccatctctgttaatattgatggaaacagaacctgtgactcgatgccaccgtcgaaccaaaaatttcattctggaaattgcaatggatactctgacggccgaccgaaacctggtgaagccctttgggcgattggtgatcacctctagatccgtgaaagctggctgcccccccatccgggcaagcagggccaaggtggcatcttcacattcctggaacccacccagtaacagcagcaggtatttcttctggtaaatgagagcctttcgaaaactttctgccctcaagtatttaccataaattctctttaaagtgacatgttcagaatcagggctcagagtttgaagtaaagagtcatttcttagttcagctttcagtttgtatacttcagcctctgcccttttcaaagatttctggagagtcaatttttctctgttccatacttctttttcagaggcaatgatggcttcaatgttggcaccaccattcaatgaaaacctggaagaattatctctaccagctcctgtctgtcgataccacctgatctgctcttccagcttcataaccatgttccttaagtcattcttctcttcagtcagttgactgatatgccctgtcagctcagcattttgtctcagtagtctttcagtcaatgagccacaagaagtacttggggacaccaagctgggctcttcaccttgctggccagttaatttctgtagttgtaaaataatttcatcaatattttcctgaacccaaatgaaatcttcatcatctgctgtttcaaactgtagtctctcagaggctttctggggtagaacctgtagttttgaagctacacattgaagcttttgtctgatcatttctaattcatgattacagccggttcctcctccattcatttcaatcaatttagcgtagtttgattcttttgtttctccttctattttctgttgaagaacccaatttctagttctatcactggttaagctccacgtggttggctcattaaggttctgatacagaattcttctactttctcgtttttcttctcgttctagttcttgcttctggaattcctgcatgattccttgtagtcgctgtccttcaaggtctaacttataaacttgttgtcttttctcttccagctggcgctgaagatcttccactttggactggagctcatgcatttttttctgtccctcagtgttggcctcctgttctgtctgcagtgttttcctgtgaacctgcctatctttttccatttgctgtcgtgtttgcaaagaatccagtttatatttttcagtctcatttaacaattctactatgcgactgtgtttttcctctagctgtttctgcagctctttcagtaggtcctctgagggcaagggtggccgagactgtccagtaccatcactgctctgcagctgtgcgtgcaattcccgctccctatctagggtactactcatttcccgaattcgaactttctcagattcaagaagtacctgaagctctaagtttcgaccttgttcttctgacaactgggcatcatatagcattctctgtgattctattttttgctgggattcgttcagtagttgtttctgttgttccaaaagtagatttagctgaagattcctttgtttctgactctcaagtgaaaacttcagatcctcaagttcttctttatcccgttcttcactgcgtcccaacttggctttctctttctccaaagcccactggagctctcttgattttttctgttcacttgctaatgtgtcattaagcaaatgtacttcatctgtcttatctttaacttccaacctgaaagcctccaattcttttaggtgtttatgctgtgccttgagtgttgtttctagttccaatttagtttgtgcaagctcactcttcagttcagcaaccaccattttctcagaactcagctgctcctgcagttccgttgctctgtctttcatactgctgagctccacttgcatctccagcatttgagactgcttctgctgtatattatattccaagagttcttggcttggtttctcactctcttgttctcttttcagagtaattttcctaccattcatttgtgcatgcagtgcctgaatttcagataacaaactccttctatctgctttctggaggcattccatagctgcttgatattcaacaccctgttcttgtattctctgttccaaacagtttagtaaaccaactgcatctgtagtacctagagctgtcagctccgtccgaaatgctgctagtaaaacactacgctcttctaagaaaacttgttgaagggcaagcagtagttcacctcgccagtctgagaagctctcatgagattgagaactatcataaacctcggcttctctttgcagttgcatctttgtaattaaatcctttagagatgagattgtattgatgtaagcttttctctcttctagccaaggttctgaaacctgctgaatagaatggtcctctccatcactatagggagactcagtgagagaaagcacctgcatgccttcattatggacagctctcagtaatccctttattttctttggaaaggaatctgttgcactttcactttcttctcctcggccttctgatgctatgtcaaatccctgactgtgtgtaagataaattccctgaccccagtctgatccagaatcactggagcatatttctctagtctggtaagcatcagaatgtgctagctcaggaattgaggatccctctttacttctcagacactgtatcactgccttcaaggtaccacattcctctttcagtaactgaacggcaacatagtgttccctctttaaggtttcagtttctgaaatatgtctggattccatgtccaaaatttcagcagcatgtagttcttgcatcttctcaattttttcagtaaactgactgattatttcagtaacttcttctgaggaacattcactctgtaaattaatttgtattcctgcatttttaacaagaatttgtggagtctgattgctgctactgatcttcagagtcccatctgtctgggatgcaatgctcttactcagttttataggaagtggctcaaacatgcaggcctttttgctttcttgtacctcagtctcatcttctttttctaaaatggacaatttctcttttgcctctgcgaggtgatccctaacttggcttaagtctttctgaagagatgtcatatttgtttcttttaccaaaagctcttcttgaagtttttcagccttttctttataactggcaagttctgctttggtagccactgattcagctctaagagcctcgagttcattaaaaaatccactttcttcattgctatgaaatagctcagtagttgtcttgagaacttcaacatcttgagggcttcttttcttttctttctctctctgttttttctcattgccctccaatagcttctgtagttctagcagcttcttttctttttctaaaacatttttttctgcaatttctacttgttctttttctaaaatcaaactagtatgcatttcaacaacctggctttctaattctgatattctcaaggttaatgctgatatatctgaccccaactcatcttctcttagttgatttaaattctgaatatttgttctttcaggttctgatgaaattgtttgattatcttgacagaattttgcatattcctgaactgcctcaagttggatttgactgacaagagcagcagccactttttcttcaactattttctgtaggtttacaatcttcttttgaagcatttctgtttcaaactggccttgttcttgcatgtcttttatttgtttataacactgggtaagttctaagtcctttgcactaacagtgctctcaagttgtagcaaccttgtttccaaattaattatggaacctttgccattttcttcaaaagatttgaagtatgtctgattttctagggatttaagagcatcctctgtaaggactacttctagttcaggtttgtctttgctcagatgatctatagccacgttaacactattctctggtatgctttgaatcttttccacactttcacgttctctctttaagctgaataattcctgtgttagctgattcattttaaaattggtttctttaagtacatttttcatgaaggtcatttcttcattagcggtttctacttgctgttccaaggccagcttttcagctataaccacatccaattgatgttttaaactgtctgcttcttctgagagggaatgagcattcattgatgtcttctgtccaatatttgccaattcctgttgaagtttttcaatcacttcattgagctgctctatttcttcttctctatttctcttcacacattcttgatcactcatcaaacattctatttgggtttcaagatcccttatcagttcatttttttcttcaataaccttgttatctgttgtaattttaagttgctgctggagtttcgtaacttgttcatttaattggtcaatttctacctctttttcctgtattatttgagcaaatttcccaaatagcacatgttggtcttgagtagacatggcatcagattcctttatggcaagtcccagtttctccatgtcatccttaaataatttgttttcctgttcaagttcttgtaggcgggtagtagattcctttttctgtatttctaattgcatatgtaattgttgaacttcttcattcttattttccagttcttctctaaactgttctaattgctcttctaagtttgtaatctctttttcctttctgtctatggcatctcgttcagcctgcaattgtacttctagggacaattctggtttagcttctacagctccaaagtgttttcggtcctctaccttttgaaaagtatctgcactcacaagaagcgcctgctccagttctcttactctgaactccagtttctctatttcttcattcctttcttgtatatccctttgaagctgctctttagagagcaaaagctcactgcatttgtctgttttttctttcagatgatttgctaactgttcaacctctctagtttgatgttcactgataggctggaatcgaggaacaaccttaagttgctgttctagtttctgtatttcctgttggaatacatctctctcatgttctctgtcaatggcttgctcatctaaaaattttctcattttttctaactgcttttccaatgcttggttttgctgtcttaaatccattagttcagtatttttttcttgttccagctctataaacctactgacttgttcttccacatctatttctagagctttcacttgtttttgaaggtcatcacgtactttttcagcttgacattgtacttctagtttttccttcattaatttttctgtctcctgtagtaattctgctcctggtgctgcatcgactgcagcatctactagtcgttgttcaactgggcctgcctctgctttcatagcttccttttgtctggacagtaattctctttcttcttggatctgctgttgctctgcctccaattcttgcaacctgttacttgcacataacaactcctgctcaagacgatctattatatcagttttttcctgaatttgcctttcaaaaagagttttttcatctgcatagccatcaatgacgccctcagccttactgagctccacagctagctgttctctggccctggactcctcatgaaggcgctctcgaagttcctcttggcacttaagggactctgttgcttcttgtttctgtctaaatgactcacgcatcaactctgtctgtgtcactttcgcatgttcaagctgactgctagtttcacttatggcttctaggagtttttcaactgctgcttgtagtcgagagctaatgttcagcataagttcttcattttcagggtctatttcagttccagcaaaaccactcctcacaagtcgttgtgacagctctgttccttcctcagttacttttgaccacatgttaatgtcatttcttggcatatcacttccagaataagagggaatggattcatctgtaactcttgtatgttcctcatggacacatgactttacagatgcctctgcttctgacctccaaattaggctggcagatgactggcttttactagatctatctagaatcccaaggacatggcgaccaattgtttcttcaacagctgctgttgtctttacaacttctaagaggatcttcaaaagtctattattagctttctggagtgcatacactgtctttcttgtttgagttccatactgactgcgttccatactgatgatccaatggggaagccaaaatcttaggggccaaattcctccatgcaagctttcattagacaaaatctcaggaggcacatcttcaggttttctgtctaattccttttctttaaatgtttgttcttcaacttctccttggttttcatttccattctgggctaattgtctattaagtctcttaatctcttcttgtagctgttcctggtcttctcgctgtctctccatttgccgcatatgtgcttgccttaacaattccgttgcctgttgatgttcttggtattgtcgtacaagttcctgtctcatatcttccaactgttcttcattcaacattagttgtctagaagcatccatgcttgacactgaaatctcatcatgaatagactgtctaactataaatgttttatctttggagaacatttcttctgaaatagtcagcacacagtcctttgattctggtatatcatggggatcactatttgataataaaatttcctttccatgttctcctaactctttactaagtggtttaaattcttctttaaatttcacatccactgtctcaaaagtctgaaaaccaatttgatcctgtgataatttcatttcattaaaataatgttgttcttgctgacacacagcatgtgcttgctttgatgatgcagtattttcttttcccccagatattctagacagttcagtttgttgagcaaatgctatactcattgacacaataaccttagctacttcttcttctaattgttcttggtattgtttttcaagcaacttaacgatatttgtttcctctttcactccaaattcaccagaaaactctattgtaccatcaatattctttttcacacaacttccagggtacattgttctctgtgcatcagattctgtaattaccaccgaatcaacaggtaagcttggcggaaccgtggactcactaacagcttgaagcctcttctgtaaacagtggatctctgcctcatagttttgttcagtttctttcaactgttgctgcaaagaggatatgaggctttctaattcttgaacttgttcttcaagtttagttttttcaagatcttgcagagaagataacttgcttttatgattgacatcaatgtcttccaaattggtcatctgagaatggattgataaaaactctgtttcctcttttggaaggttttcttctccaaattcaagtttcataccatctgtctgctgtccccagatcttgcttagtcgtgtttgaagtaccaagagtttgttgtattcttctgttactttgttgagaagagtgtgcatattttcttgaaagtcttgaacttcatatctataatcttgtaattctggatcttcattttcagaaatgtaatcaccagaattctctttgtcttctgcatttacttcacattttaaagcaggagtataatattcaccaaggacactgcataaagtctgtaaaaaataagaacattcttcagacactgccttttgaagttttccaatgagcagatgtaaaggctttccttcatcacctgtttcttgtgttttcatagtctgtagttctaactggtgtattttctgaagttccttgatcttttcctcttgagcaaaaataagctcttctttaagactgcaaagagctttatctttttcattttccatatattcacgaacctgatccacatgagttgaataaaccagagagaggcaaatgcgttgggcttccatctgtagccttaaatcattctgttctgatttaagtacattgagttctttctgaagtttatcattttcacttggttgagttgctctaagtgatgattcctttgttacagatggtaagtgatccaaaatcaactgttcttgcttactttcttctccaacagtcatattttcaaaagaaactttatcttccaccattatttttgattcttcaccaaaacttttatttactttagaaactgatccttcagcacccctgcttgtcatggtcacaactccatctaataaagagcttacttgagtatcacatgactgtacattttctgccctgttgtggttaataatgatttctagctctctacatctcaatgaaacttgttctttctcttgctttaaagatttaacttcttcatttagaaaactaatctcaccatgtttctgtttcaattgttcagaaagatcagacagtctctgtgacagctctaatttctctcgcttggttacctcaagtttttccatgagttctgttgtatccttttcaacaacctcacccatttccaatgtttctgctacaaaagttttgtcttcatcaaagacagaacttttcattttcactgtagttggatttattctttgcaaatgaagctcttcattaagtgctttaagtttacttttatactctaattcctgtttatttttactgtcttctaaatcatcttttactttgagaaggcaagcatactcctcttgtaactcttgatagttaacttcaaagtttttttcagcaaatgaaaaagtgttcctttgcttttcaatctcttcatttagctgaatacattgttgtttgaggtcctcattttcctctataagtatttctatttctttttcccacacagagtctttggatttggacttaatggagtctaagaaaatcaatctttcttcttggctaacaggagtatgtattttcaacatgtcttcaagggttttcttttcatctttaagaatgctattctctgcttcaagttgtgcaaatttttcttgaagatcattctctttttccttcatctgtttttctaacaattctgttttaagttgtaattcttgaacttcttgttcaagtgtacccttttctttttcttcttgtctgagtatttcaatttctttttgaagttcattgatttgaagagtcatttcttctgactttgaatttacaagagactgctgtaaatcttttagctttgaaatttccaaaattaattgattctgcttagttatcaaattgtccttttcaaactgcatggtttctatcttttgactcatttcattctgtaaaccatctatctgctgtttatagtgaatgcctaaattatctttaagtttttcaatatttattcgatgttcaatttctaaatcttccttcagtttggaaagctcttcttcgtgactaaatagaagctgtgttctcagcctctctaattcagcttcttgtgattcagccattctgtctaacacagcattcttttctttttctaacatttcaagttttatcttgtaatttgtaacttctgcttcatgttttaattctagttcctttctggattcagatgcagaaacaatctcagctttcaaatcttccactgtactaagggacttatgtgcttcattaagtttactttcttgttcagctattgtctgtctagctctctgaatctgttcccttgaaaagctcaattcttcaacaaggtcttcaagctgtctctgtagagcacacttttcttctaaaattagtcctagttcttccttgagtttttccttttgagagttagtatcttgcaattttatattcagttcatttattgccacattcattaactttatctgatcttcattaactgtaatatttgaatatgaccttaaagcattctccatttctcccttatgccgtgttttcatttcctccatctgtgccatgtgttgtcttattaattcttgtttcatttgcactatctgctgcccatacatctcatccagctctgcccggagttgttctaactttctttgtgtttcttgttccattcgttgtactatatcagtttcgaactggctgtctttatgatttctcttctgaagttcttcgactgtccccattaactgttttatttcttcagaagactgtctttctttttgcttagaattagtcagctctaatttcatgttttttatttcttggttcttttgcacaatctgttcttgtaattctcctagtaatttatcagcagttgttaatttatcctttagctcaagagttttcttttcttcttctattatttttgtgtttaattcttcaatgattgtctccttttcctgtatttcttctttatttgagttttctacttttttatcttgttccatttcatatactttaattttctcttgcaagaaactaatttgcattgtgaagtcttctttctttttctgataatcttctaataagtggtcttgttcttcaagctgctgttgatgagtgaggatctgttgtttggcttgtagtaagtctgcagctgtgctactatgagtgctgtttctcagagtttcactagcctgtaattgctgaaattgaatctgtaatttttgactctgttctgtcaactctaaaaattctctcattgtctcatccttttctcttcttgcttgttgtaaattagcagtgagctgggttataatgccatctctttgtttaatggcagcttcaaattcttgtaactgctgcagtccttcagtcccataggtaaccctcatttcttccagctctctgtttagctcttcaatctcatgctgcttcccagccaactcactttccatcatctctagatgagtcggactgtcttgtgctccttgttcagaataagaatcatcaacaccaaattcttcttcccttaataaatttgtaggctttcctgttctcatcacaaaactgcaaccatttacctctgaactgcagtcatctgctgtggttgaaatttcactttccagttccacagagaagccctgctcatgactggttatttctccactatgtagagttctcattattgtagattcaggaatcacagttgattctactctctgagaactatttatgtacatttcattacactgtgattgatcaatattcaaatcatggtgtgctgacacatcatgtttactgcttgacgtttttctcttttttttctgcttcttggaaggactctgcccatccgactgagcttttctttgtcgaaactgggcaagcttggctttgccggcctccagcttcttctgtctctcctcgtcctccatggcctctgcaaggaaggcaggggaaaacaggggttgaggggtggttggggatagaaaggaaaggtcgatttggacggaggtgggacggcaagctccacggcctagagagccgattcggtccggcgctcccccgcccgaagtggaagcagtctccgcgctcactggcggatcgtcctcagccgcacgggaagcgccgtcaccgccgccgccgccgccatcttcgtctccacgta

SEQ ID NO: 14128 - RNA, 11512 nt, Homo sapiens
  source 1..11512: mol_type = other RNA
gctgggattacaggcatgagccaccgcacctggccttccctgcttcctctctagaatccaattagggatgtttgttactactcatattgattaaaacagttaacaaacttttttctttttaaaatgtgagatcagtgaactctggttttaagataatctgaaacaaggtccttgggagtaataaaattggtcacattctgtaaagcacattctgtttaggaatcaacttatctcaaattgtaactcggggcctaactatatgagatggctgaaaaaataccacatcgtctgttttcactaggtgatgccaaaatattttgctttatgtatattacagttctttttaaaacactggaagactcatgttaaactctaattgtgaaggcagaatctctgctaatttttcagattaaaattctctttgaaaaaatacagtctgtattcatgaattgtaaaatatgtgcttcagtgagcagagttagggaatccaggaacttgggtggggaaaaattacatctttatttgcactaataatttctaactgcaatttagtatttatttcaattatgaatttgggcagcattttattagcagtatccatgattttgtcaatagaaatctcagatattttcatattacagatgttacagatttcttgaagtatctagttacgaccccgagataaggctagtctaatgtttagtgaatagttttagacttcttaacagatttcatttttaatcacagactaattaattattgagatgcataaacaagtgtgattgcagaggcctactatcataaggaggcgtggtggtcaaacaatggcactgaactcagcttgatcagatcatttgtccatctgtttttttctccactgtctcttagagcagaatagccttgaatggcaagccatgctagctgaaaaaggtttttacccacaacctgccccttcaactaactgctttagagtacgtttgctatttttagaattcctcttattggaacccagcttctaatgtggaaaatttaagtatagttggctccttttatttgtgggttctgtatcctctgattcaaccaactgcaggttcaaaatactaaaaataaaaccccacaataaaaaaatacagtattagcaactatttacataatgttcacattgtattaggtatcaaataatctggagatgatttgaagtacacaggaggatgtatgtagactatctgcaaatagcacattgttttataagagacttaagcattcgcggactgtaatatccaagggggatcctggaactaatcccccacacatgccgagggatgactgaaattagaaatgttcaagcatgtacaactttctaccatgcctgtttgtgttggtataaatcatggaacatcaaataataagacaaaatcctccaggtgtaagcatcaaatactagtcctcttgctgttttagtgagttgccatgttattgaggaggactccagatgagaaataacattgcgatctgtattatctctgtgagagcctcccagtctgaatttggcttggacaacagggatactgtttaattcggctgcaatgtgattaagatcttttgagttaatgatttcttcatctttttagtgggccatggatttgtgagaacacatctttggaaacaagtaacactaactgtaatatagtaaatactgattaatcatgaaataccaatatagcttttaaaaaacactatgtagatgtaaagttgatacaaagacacatggaaaactttcaacagtattaactctaagattaggacaactttctctgaatctctcactcctacatatttgacataagtaatgagatgctatgtaccaagaactatggctcagttaaaaatgaagaaggttcaaatacagtgtggtgaaaatggtgaagtcatttttatttcagtacttgacaaaataccccataaaattcaaaacttctaccattatacaaaaataggtctctacaagtgatattatctgtcttcatcaccagtagaatatattaggcaaaacatgtaacttcagtagccttataagaaaagtgcaggacacctcgagctacacattcagcagtattgtaatgcgtaaaagtttaatcttttcacccatttgataaatacacaaggtttataatttaatgttttaaattagcattccacaaatatacaggtaattcaataattattgtgcatgaatacatacacaatgcttatatatacaaattccagtttgttttcatgtgctggcaagggatttgtatacaatcataagctgtgttcatattggtcccattgaatattcacaatacaaaagcacaaaagaaccattgatttacaaaaggaaatctatttaaaatcacttcaattaatgatgtttcaaaggattatcttctcatgccagcatgaaattgagtagttgaacctatgagagaaaaacaggaaattcaactgatttcaaattacattgctacctgtatcagacccaccagagttcacacaaaggaaattattattattctccatttttttaaagccctttttttccttaaaatgtcctcttcatacttaaactgagtctctccccactacccccaaggtggagtgttactctgttgcccaggctggaattcagtggtgtgatcttggctcactgcaacccccgcctcctgggttcaagtgattctcctgcctcagcctcctgagtagctgggactatccacacatgccaccatgtccagcaaatttttgtatttttagtggagacggggtttcaccatgttggccaggctagtctcgaactggttggtcttgaactcctgacctagtgatccgcctgcctcggccgcccaaagtgctgggattacaggcatgagccaccgcgcccagcccatatacttaagctgacttttaagagattttgaatatatatgtaaaaatcaccatgactggctctatggcaaggtaggtgagactaatatttagagtttttttaaagtgctctcaaagttggatgttctatacctcatacatttttgaaaaatcttttggtcttcaaaatctgggtcttgtgaaatttggatgctcaaaacaaaacaagcctaggcaaaccaacaaactcagctatgataataaaagtttcctattactacaagatgcttgggtgtaaacaaatgatttcttgaaggaagagataaactactcaatgattcaaagtctctgaatcaggagtgaactgaagtgagatagggaaaagaggttttccttccatgaacagggaatccacctttattttaaagtatgacttgttttttgtttttgaacaaagaaaaaataatccttacaaagtattttaaatgggatagtttttttcgatgatacataaaagcacaatatagtagcagggataatggttacattaagtgcttaaagtaagtgcttcctccttaactccacccgatttgcatgccttaccactttcttttttttttttttttctttgagacagggtctcgctctgctgcccaggctggagtgctgcggcacggccttaccactttctgccatgcgctacttaggaatacgttctccagttaggctctgtagactcagagtaccttgcacactggtgctcattgtgcattttgtgtcatcagtccgctgaatgaacatagtaggaaatcatttttgggaggagtgggatctggggtgataaatcatattttcacttaaattatttaaagtcagtttctctgctggttacaagagtttaagctttggctaacttaataattagctcatgcactaaactggaagctttgattatcctaatgagtgtgaaagaatttcaaagaaaggggagctgtgggtctcgcactgtggtgctgccaagatgtggttaaactcagagcacctgactgtatagttccaagtcgtctttgcagtgcctctagccgagtgatataatctgttagggctctgtcaggatcgtaattctgaagctgagaacatgctaaagaaccaggattgaaatcagctggagtgcctgggtacctattctgaaatggtaaaggggacctaatatagtccagatctgatcttgagcgatacgtagtatgtcttggttctccatataactccagcccaccagaagaatgataaaatgagtcagtcttttctgcaccttgattcagtccaaagccatctctgttaatattgatggaaacagaacctgtgactcgatgccaccgtcgaaccaaaaatttcattctggaaattgcaatggatactctgacggccgaccgaaacctggtgaagccctttgggcgattggtgatcacctctagatccgtgaaagctggctgcccccccatccgggcaagcagggccaaggtggcatcttcacattcctggaacccacccagtaacagcagcaggtatttcttctggtaaatgagagcctttcgaaaactttctgccctcaagtatttaccataaattctctttaaagtgacatgttcagaatcagggctcagagtttgaagtaaagagtcatttcttagttcagctttcagtttgtatacttcagcctctgcccttttcaaagatttctggagagtcaatttttctctgttccatacttctttttcagaggcaatgatggcttcaatgttggcaccaccattcaatgaaaacctggaagaattatctctaccagctcctgtctgtcgataccacctgatctgctcttccagcttcataaccatgttccttaagtcattcttctcttcagtcagttgactgatatgccctgtcagctcagcattttgtctcagtagtctttcagtcaatgagccacaagaagtacttggggacaccaagctgggctcttcaccttgctggccagttaatttctgtagttgtaaaataatttcatcaatattttcctgaacccaaatgaaatcttcatcatctgctgtttcaaactgtagtctctcagaggctttctggggtagaacctgtagttttgaagctacacattgaagcttttgtctgatcatttctaattcatgattacagccggttcctcctccattcatttcaatcaatttagcgtagtttgattcttttgtttctccttctattttctgttgaagaacccaatttctagttctatcactggttaagctccacgtggttggctcattaaggttctgatacagaattcttctactttctcgtttttcttctcgttctagttcttgcttctggaattcctgcatgattccttgtagtcgctgtccttcaaggtctaacttataaacttgttgtcttttctcttccagctggcgctgaagatcttccactttggactggagctcatgcatttttttctgtccctcagtgttggcctcctgttctgtctgcagtgttttcctgtgaacctgcctatctttttccatttgctgtcgtgtttgcaaagaatccagtttatatttttcagtctcatttaacaattctactatgcgactgtgtttttcctctagctgtttctgcagctctttcagtaggtcctctgagggcaagggtggccgagactgtccagtaccatcactgctctgcagctgtgcgtgcaattcccgctccctatctagggtactactcatttcccgaattcgaactttctcagattcaagaagtacctgaagctctaagtttcgaccttgttcttctgacaactgggcatcatatagcattctctgtgattctattttttgctgggattcgttcagtagttgtttctgttgttccaaaagtagatttagctgaagattcctttgtttctgactctcaagtgaaaacttcagatcctcaagttcttctttatcccgttcttcactgcgtcccaacttggctttctctttctccaaagcccactggagctctcttgattttttctgttcacttgctaatgtgtcattaagcaaatgtacttcatctgtcttatctttaacttccaacctgaaagcctccaattcttttaggtgtttatgctgtgccttgagtgttgtttctagttccaatttagtttgtgcaagctcactcttcagttcagcaaccaccattttctcagaactcagctgctcctgcagttccgttgctctgtctttcatactgctgagctccacttgcatctccagcatttgagactgcttctgctgtatattatattccaagagttcttggcttggtttctcactctcttgttctcttttcagagtaattttcctaccattcatttgtgcatgcagtgcctgaatttcagataacaaactccttctatctgctttctggaggcattccatagctgcttgatattcaacaccctgttcttgtattctctgttccaaacagtttagtaaaccaactgcatctgtagtacctagagctgtcagctccgtccgaaatgctgctagtaaaacactacgctcttctaagaaaacttgttgaagggcaagcagtagttcacctcgccagtctgagaagctctcatgagattgagaactatcataaacctcggcttctctttgcagttgcatctttgtaattaaatcctttagagatgagattgtattgatgtaagcttttctctcttctagccaaggttctgaaacctgctgaatagaatggtcctctccatcactatagggagactcagtgagagaaagcacctgcatgccttcattatggacagctctcagtaatccctttattttctttggaaaggaatctgttgcactttcactttcttctcctcggccttctgatgctatgtcaaatccctgactgtgtgtaagataaattccctgaccccagtctgatccagaatcactggagcatatttctctagtctggtaagcatcagaatgtgctagctcaggaattgaggatccctctttacttctcagacactgtatcactgccttcaaggtaccacattcctctttcagtaactgaacggcaacatagtgttccctctttaaggtttcagtttctgaaatatgtctggattccatgtccaaaatttcagcagcatgtagttcttgcatcttctcaattttttcagtaaactgactgattatttcagtaacttcttctgaggaacattcactctgtaaattaatttgtattcctgcatttttaacaagaatttgtggagtctgattgctgctactgatcttcagagtcccatctgtctgggatgcaatgctcttactcagttttataggaagtggctcaaacatgcaggcctttttgctttcttgtacctcagtctcatcttctttttctaaaatggacaatttctcttttgcctctgcgaggtgatccctaacttggcttaagtctttctgaagagatgtcatatttgtttcttttaccaaaagctcttcttgaagtttttcagccttttctttataactggcaagttctgctttggtagccactgattcagctctaagagcctcgagttcattaaaaaatccactttcttcattgctatgaaatagctcagtagttgtcttgagaacttcaacatcttgagggcttcttttcttttctttctctctctgttttttctcattgccctccaatagcttctgtagttctagcagcttcttttctttttctaaaacatttttttctgcaatttctacttgttctttttctaaaatcaaactagtatgcatttcaacaacctggctttctaattctgatattctcaaggttaatgctgatatatctgaccccaactcatcttctcttagttgatttaaattctgaatatttgttctttcaggttctgatgaaattgtttgattatcttgacagaattttgcatattcctgaactgcctcaagttggatttgactgacaagagcagcagccactttttcttcaactattttctgtaggtttacaatcttcttttgaagcatttctgtttcaaactggccttgttcttgcatgtcttttatttgtttataacactgggtaagttctaagtcctttgcactaacagtgctctcaagttgtagcaaccttgtttccaaattaattatggaacctttgccattttcttcaaaagatttgaagtatgtctgattttctagggatttaagagcatcctctgtaaggactacttctagttcaggtttgtctttgctcagatgatctatagccacgttaacactattctctggtatgctttgaatcttttccacactttcacgttctctctttaagctgaataattcctgtgttagctgattcattttaaaattggtttctttaagtacatttttcatgaaggtcatttcttcattagcggtttctacttgctgttccaaggccagcttttcagctataaccacatccaattgatgttttaaactgtctgcttcttctgagagggaatgagcattcattgatgtcttctgtccaatatttgccaattcctgttgaagtttttcaatcacttcattgagctgctctatttcttcttctctatttctcttcacacattcttgatcactcatcaaacattctatttgggtttcaagatcccttatcagttcatttttttcttcaataaccttgttatctgttgtaattttaagttgctgctggagtttcgtaacttgttcatttaattggtcaatttctacctctttttcctgtattatttgagcaaatttcccaaatagcacatgttggtcttgagtagacatggcatcagattcctttatggcaagtcccagtttctccatgtcatccttaaataatttgttttcctgttcaagttcttgtaggcgggtagtagattcctttttctgtatttctaattgcatatgtaattgttgaacttcttcattcttattttccagttcttctctaaactgttctaattgctcttctaagtttgtaatctctttttcctttctgtctatggcatctcgttcagcctgcaattgtacttctagggacaattctggtttagcttctacagctccaaagtgttttcggtcctctaccttttgaaaagtatctgcactcacaagaagcgcctgctccagttctcttactctgaactccagtttctctatttcttcattcctttcttgtatatccctttgaagctgctctttagagagcaaaagctcactgcatttgtctgttttttctttcagatgatttgctaactgttcaacctctctagtttgatgttcactgataggctggaatcgaggaacaaccttaagttgctgttctagtttctgtatttcctgttggaatacatctctctcatgttctctgtcaatggcttgctcatctaaaaattttctcattttttctaactgcttttccaatgcttggttttgctgtcttaaatccattagttcagtatttttttcttgttccagctctataaacctactgacttgttcttccacatctatttctagagctttcacttgtttttgaaggtcatcacgtactttttcagcttgacattgtacttctagtttttccttcattaatttttctgtctcctgtagtaattctgctcctggtgctgcatcgactgcagcatctactagtcgttgttcaactgggcctgcctctgctttcatagcttccttttgtctggacagtaattctctttcttcttggatctgctgttgctctgcctccaattcttgcaacctgttacttgcacataacaactcctgctcaagacgatctattatatcagttttttcctgaatttgcctttcaaaaagagttttttcatctgcatagccatcaatgacgccctcagccttactgagctccacagctagctgttctctggccctggactcctcatgaaggcgctctcgaagttcctcttggcacttaagggactctgttgcttcttgtttctgtctaaatgactcacgcatcaactctgtctgtgtcactttcgcatgttcaagctgactgctagtttcacttatggcttctaggagtttttcaactgctgcttgtagtcgagagctaatgttcagcataagttcttcattttcagggtctatttcagttccagcaaaaccactcctcacaagtcgttgtgacagctctgttccttcctcagttacttttgaccacatgttaatgtcatttcttggcatatcacttccagaataagagggaatggattcatctgtaactcttgtatgttcctcatggacacatgactttacagatgcctctgcttctgacctccaaattaggctggcagatgactggcttttactagatctatctagaatcccaaggacatggcgaccaattgtttcttcaacagctgctgttgtctttacaacttctaagaggatcttcaaaagtctattattagctttctggagtgcatacactgtctttcttgtttgagttccatactgactgcgttccatactgatgatccaatggggaagccaaaatcttaggggccaaattcctccatgcaagctttcattagacaaaatctcaggaggcacatcttcaggttttctgtctaattccttttctttaaatgtttgttcttcaacttctccttggttttcatttccattctgtgtttgcgtactgctgttgcgcagctcacaacacagcttctctcttccagctaaagacagctgctttagtgcttccagctcctctaaaagcaccctctctctctctgaaaccaggttttcattatctatggaggatctctgggctaattgtctattaagtctcttaatctcttcttgtagctgttcctggtcttctcgctgtctctccatttgccgcatatgtgcttgccttaacaattccgttgcctgttgatgttcttggtattgtcgtacaagttcctgtctcatatcttccaactgttcttcattcaacattagttgtctagaagcatccatgcttgacactgaaatctcatcatgaatagactgtctaactataaatgttttatctttggagaacatttcttctgaaatagtcagcacacagtcctttgattctggtatatcatggggatcactatttgataataaaatttcctttccatgttctcctaactctttactaagtggtttaaattcttctttaaatttcacatccactgtctcaaaagtctgaaaaccaatttgatcctgtgataatttcatttcattaaaataatgttgttcttgctgacacacagcatgtgcttgctttgatgatgcagtattttcttttcccccagatattctagacagttcagtttgttgagcaaatgctatactcattgacacaataaccatcgataaaatctatgttctttttgaaggctcaaagggaatataaaccaagataatcttccagataagctataagccta

SEQ ID NO: 14129 - RNA, 15592 nt, Homo sapiens
  source 1..15592: mol_type = other RNA
gctgggattacaggcatgagccaccgcacctggccttccctgcttcctctctagaatccaattagggatgtttgttactactcatattgattaaaacagttaacaaacttttttctttttaaaatgtgagatcagtgaactctggttttaagataatctgaaacaaggtccttgggagtaataaaattggtcacattctgtaaagcacattctgtttaggaatcaacttatctcaaattgtaactcggggcctaactatatgagatggctgaaaaaataccacatcgtctgttttcactaggtgatgccaaaatattttgctttatgtatattacagttctttttaaaacactggaagactcatgttaaactctaattgtgaaggcagaatctctgctaatttttcagattaaaattctctttgaaaaaatacagtctgtattcatgaattgtaaaatatgtgcttcagtgagcagagttagggaatccaggaacttgggtggggaaaaattacatctttatttgcactaataatttctaactgcaatttagtatttatttcaattatgaatttgggcagcattttattagcagtatccatgattttgtcaatagaaatctcagatattttcatattacagatgttacagatttcttgaagtatctagttacgaccccgagataaggctagtctaatgtttagtgaatagttttagacttcttaacagatttcatttttaatcacagactaattaattattgagatgcataaacaagtgtgattgcagaggcctactatcataaggaggcgtggtggtcaaacaatggcactgaactcagcttgatcagatcatttgtccatctgtttttttctccactgtctcttagagcagaatagccttgaatggcaagccatgctagctgaaaaaggtttttacccacaacctgccccttcaactaactgctttagagtacgtttgctatttttagaattcctcttattggaacccagcttctaatgtggaaaatttaagtatagttggctccttttatttgtgggttctgtatcctctgattcaaccaactgcaggttcaaaatactaaaaataaaaccccacaataaaaaaatacagtattagcaactatttacataatgttcacattgtattaggtatcaaataatctggagatgatttgaagtacacaggaggatgtatgtagactatctgcaaatagcacattgttttataagagacttaagcattcgcggactgtaatatccaagggggatcctggaactaatcccccacacatgccgagggatgactgaaattagaaatgttcaagcatgtacaactttctaccatgcctgtttgtgttggtataaatcatggaacatcaaataataagacaaaatcctccaggtgtaagcatcaaatactagtcctcttgctgttttagtgagttgccatgttattgaggaggactccagatgagaaataacattgcgatctgtattatctctgtgagagcctcccagtctgaatttggcttggacaacagggatactgtttaattcggctgcaatgtgattaagatcttttgagttaatgatttcttcatctttttagtgggccatggatttgtgagaacacatctttggaaacaagtaacactaactgtaatatagtaaatactgattaatcatgaaataccaatatagcttttaaaaaacactatgtagatgtaaagttgatacaaagacacatggaaaactttcaacagtattaactctaagattaggacaactttctctgaatctctcactcctacatatttgacataagtaatgagatgctatgtaccaagaactatggctcagttaaaaatgaagaaggttcaaatacagtgtggtgaaaatggtgaagtcatttttatttcagtacttgacaaaataccccataaaattcaaaacttctaccattatacaaaaataggtctctacaagtgatattatctgtcttcatcaccagtagaatatattaggcaaaacatgtaacttcagtagccttataagaaaagtgcaggacacctcgagctacacattcagcagtattgtaatgcgtaaaagtttaatcttttcacccatttgataaatacacaaggtttataatttaatgttttaaattagcattccacaaatatacaggtaattcaataattattgtgcatgaatacatacacaatgcttatatatacaaattccagtttgttttcatgtgctggcaagggatttgtatacaatcataagctgtgttcatattggtcccattgaatattcacaatacaaaagcacaaaagaaccattgatttacaaaaggaaatctatttaaaatcacttcaattaatgatgtttcaaaggattatcttctcatgccagcatgaaattgagtagttgaacctatgagagaaaaacaggaaattcaactgatttcaaattacattgctacctgtatcagacccaccagagttcacacaaaggaaattattattattctccatttttttaaagccctttttttccttaaaatgtcctcttcatacttaaactgagtctctccccactacccccaaggtggagtgttactctgttgcccaggctggaattcagtggtgtgatcttggctcactgcaacccccgcctcctgggttcaagtgattctcctgcctcagcctcctgagtagctgggactatccacacatgccaccatgtccagcaaatttttgtatttttagtggagacggggtttcaccatgttggccaggctagtctcgaactggttggtcttgaactcctgacctagtgatccgcctgcctcggccgcccaaagtgctgggattacaggcatgagccaccgcgcccagcccatatacttaagctgacttttaagagattttgaatatatatgtaaaaatcaccatgactggctctatggcaaggtaggtgagactaatatttagagtttttttaaagtgctctcaaagttggatgttctatacctcatacatttttgaaaaatcttttggtcttcaaaatctgggtcttgtgaaatttggatgctcaaaacaaaacaagcctaggcaaaccaacaaactcagctatgataataaaagtttcctattactacaagatgcttgggtgtaaacaaatgatttcttgaaggaagagataaactactcaatgattcaaagtctctgaatcaggagtgaactgaagtgagatagggaaaagaggttttccttccatgaacagggaatccacctttattttaaagtatgacttgttttttgtttttgaacaaagaaaaaataatccttacaaagtattttaaatgggatagtttttttcgatgatacataaaagcacaatatagtagcagggataatggttacattaagtgcttaaagtaagtgcttcctccttaactccacccgatttgcatgccttaccactttcttttttttttttttttctttgagacagggtctcgctctgctgcccaggctggagtgctgcggcacggccttaccactttctgccatgcgctacttaggaatacgttctccagttaggctctgtagactcagagtaccttgcacactggtgctcattgtgcattttgtgtcatcagtccgctgaatgaacatagtaggaaatcatttttgggaggagtgggatctggggtgataaatcatattttcacttaaattatttaaagtcagtttctctgctggttacaagagtttaagctttggctaacttaataattagctcatgcactaaactggaagctttgattatcctaatgagtgtgaaagaatttcaaagaaaggggagctgtgggtctcgcactgtggtgctgccaagatgtggttaaactcagagcacctgactgtatagttccaagtcgtctttgcagtgcctctagccgagtgatataatctgttagggctctgtcaggatcgtaattctgaagctgagaacatgctaaagaaccaggattgaaatcagctggagtgcctgggtacctattctgaaatggtaaaggggacctaatatagtccagatctgatcttgagcgatacgtagtatgtcttggttctccatataactccagcccaccagaagaatgataaaatgagtcagtcttttctgcaccttgattcagtccaaagccatctctgttaatattgatggaaacagaacctgtgactcgatgccaccgtcgaaccaaaaatttcattctggaaattgcaatggatactctgacggccgaccgaaacctggtgaagccctttgggcgattggtgatcacctctagatccgtgaaagctggctgcccccccatccgggcaagcagggccaaggtggcatcttcacattcctggaacccacccagtaacagcagcaggtatttcttctggtaaatgagagcctttcgaaaactttctgccctcaagtatttaccataaattctctttaaagtgacatgttcagaatcagggctcagagtttgaagtaaagagtcatttcttagttcagctttcagtttgtatacttcagcctctgcccttttcaaagatttctggagagtcaatttttctctgttccatacttctttttcagaggcaatgatggcttcaatgttggcaccaccattcaatgaaaacctggaagaattatctctaccagctcctgtctgtcgataccacctgatctgctcttccagcttcataaccatgttccttaagtcattcttctcttcagtcagttgactgatatgccctgtcagctcagcattttgtctcagtagtctttcagtcaatgagccacaagaagtacttggggacaccaagctgggctcttcaccttgctggccagttaatttctgtagttgtaaaataatttcatcaatattttcctgaacccaaatgaaatcttcatcatctgctgtttcaaactgtagtctctcagaggctttctggggtagaacctgtagttttgaagctacacattgaagcttttgtctgatcatttctaattcatgattacagccggttcctcctccattcatttcaatcaatttagcgtagtttgattcttttgtttctccttctattttctgttgaagaacccaatttctagttctatcactggttaagctccacgtggttggctcattaaggttctgatacagaattcttctactttctcgtttttcttctcgttctagttcttgcttctggaattcctgcatgattccttgtagtcgctgtccttcaaggtctaacttataaacttgttgtcttttctcttccagctggcgctgaagatcttccactttggactggagctcatgcatttttttctgtccctcagtgttggcctcctgttctgtctgcagtgttttcctgtgaacctgcctatctttttccatttgctgtcgtgtttgcaaagaatccagtttatatttttcagtctcatttaacaattctactatgcgactgtgtttttcctctagctgtttctgcagctctttcagtaggtcctctgagggcaagggtggccgagactgtccagtaccatcactgctctgcagctgtgcgtgcaattcccgctccctatctagggtactactcatttcccgaattcgaactttctcagattcaagaagtacctgaagctctaagtttcgaccttgttcttctgacaactgggcatcatatagcattctctgtgattctattttttgctgggattcgttcagtagttgtttctgttgttccaaaagtagatttagctgaagattcctttgtttctgactctcaagtgaaaacttcagatcctcaagttcttctttatcccgttcttcactgcgtcccaacttggctttctctttctccaaagcccactggagctctcttgattttttctgttcacttgctaatgtgtcattaagcaaatgtacttcatctgtcttatctttaacttccaacctgaaagcctccaattcttttaggtgtttatgctgtgccttgagtgttgtttctagttccaatttagtttgtgcaagctcactcttcagttcagcaaccaccattttctcagaactcagctgctcctgcagttccgttgctctgtctttcatactgctgagctccacttgcatctccagcatttgagactgcttctgctgtatattatattccaagagttcttggcttggtttctcactctcttgttctcttttcagagtaattttcctaccattcatttgtgcatgcagtgcctgaatttcagataacaaactccttctatctgctttctggaggcattccatagctgcttgatattcaacaccctgttcttgtattctctgttccaaacagtttagtaaaccaactgcatctgtagtacctagagctgtcagctccgtccgaaatgctgctagtaaaacactacgctcttctaagaaaacttgttgaagggcaagcagtagttcacctcgccagtctgagaagctctcatgagattgagaactatcataaacctcggcttctctttgcagttgcatctttgtaattaaatcctttagagatgagattgtattgatgtaagcttttctctcttctagccaaggttctgaaacctgctgaatagaatggtcctctccatcactatagggagactcagtgagagaaagcacctgcatgccttcattatggacagctctcagtaatccctttattttctttggaaaggaatctgttgcactttcactttcttctcctcggccttctgatgctatgtcaaatccctgactgtgtgtaagataaattccctgaccccagtctgatccagaatcactggagcatatttctctagtctggtaagcatcagaatgtgctagctcaggaattgaggatccctctttacttctcagacactgtatcactgccttcaaggtaccacattcctctttcagtaactgaacggcaacatagtgttccctctttaaggtttcagtttctgaaatatgtctggattccatgtccaaaatttcagcagcatgtagttcttgcatcttctcaattttttcagtaaactgactgattatttcagtaacttcttctgaggaacattcactctgtaaattaatttgtattcctgcatttttaacaagaatttgtggagtctgattgctgctactgatcttcagagtcccatctgtctgggatgcaatgctcttactcagttttataggaagtggctcaaacatgcaggcctttttgctttcttgtacctcagtctcatcttctttttctaaaatggacaatttctcttttgcctctgcgaggtgatccctaacttggcttaagtctttctgaagagatgtcatatttgtttcttttaccaaaagctcttcttgaagtttttcagccttttctttataactggcaagttctgctttggtagccactgattcagctctaagagcctcgagttcattaaaaaatccactttcttcattgctatgaaatagctcagtagttgtcttgagaacttcaacatcttgagggcttcttttcttttctttctctctctgttttttctcattgccctccaatagcttctgtagttctagcagcttcttttctttttctaaaacatttttttctgcaatttctacttgttctttttctaaaatcaaactagtatgcatttcaacaacctggctttctaattctgatattctcaaggttaatgctgatatatctgaccccaactcatcttctcttagttgatttaaattctgaatatttgttctttcaggttctgatgaaattgtttgattatcttgacagaattttgcatattcctgaactgcctcaagttggatttgactgacaagagcagcagccactttttcttcaactattttctgtaggtttacaatcttcttttgaagcatttctgtttcaaactggccttgttcttgcatgtcttttatttgtttataacactgggtaagttctaagtcctttgcactaacagtgctctcaagttgtagcaaccttgtttccaaattaattatggaacctttgccattttcttcaaaagatttgaagtatgtctgattttctagggatttaagagcatcctctgtaaggactacttctagttcaggtttgtctttgctcagatgatctatagccacgttaacactattctctggtatgctttgaatcttttccacactttcacgttctctctttaagctgaataattcctgtgttagctgattcattttaaaattggtttctttaagtacatttttcatgaaggtcatttcttcattagcggtttctacttgctgttccaaggccagcttttcagctataaccacatccaattgatgttttaaactgtctgcttcttctgagagggaatgagcattcattgatgtcttctgtccaatatttgccaattcctgttgaagtttttcaatcacttcattgagctgctctatttcttcttctctatttctcttcacacattcttgatcactcatcaaacattctatttgggtttcaagatcccttatcagttcatttttttcttcaataaccttgttatctgttgtaattttaagttgctgctggagtttcgtaacttgttcatttaattggtcaatttctacctctttttcctgtattatttgagcaaatttcccaaatagcacatgttggtcttgagtagacatggcatcagattcctttatggcaagtcccagtttctccatgtcatccttaaataatttgttttcctgttcaagttcttgtaggcgggtagtagattcctttttctgtatttctaattgcatatgtaattgttgaacttcttcattcttattttccagttcttctctaaactgttctaattgctcttctaagtttgtaatctctttttcctttctgtctatggcatctcgttcagcctgcaattgtacttctagggacaattctggtttagcttctacagctccaaagtgttttcggtcctctaccttttgaaaagtatctgcactcacaagaagcgcctgctccagttctcttactctgaactccagtttctctatttcttcattcctttcttgtatatccctttgaagctgctctttagagagcaaaagctcactgcatttgtctgttttttctttcagatgatttgctaactgttcaacctctctagtttgatgttcactgataggctggaatcgaggaacaaccttaagttgctgttctagtttctgtatttcctgttggaatacatctctctcatgttctctgtcaatggcttgctcatctaaaaattttctcattttttctaactgcttttccaatgcttggttttgctgtcttaaatccattagttcagtatttttttcttgttccagctctataaacctactgacttgttcttccacatctatttctagagctttcacttgtttttgaaggtcatcacgtactttttcagcttgacattgtacttctagtttttccttcattaatttttctgtctcctgtagtaattctgctcctggtgctgcatcgactgcagcatctactagtcgttgttcaactgggcctgcctctgctttcatagcttccttttgtctggacagtaattctctttcttcttggatctgctgttgctctgcctccaattcttgcaacctgttacttgcacataacaactcctgctcaagacgatctattatatcagttttttcctgaatttgcctttcaaaaagagttttttcatctgcatagccatcaatgacgccctcagccttactgagctccacagctagctgttctctggccctggactcctcatgaaggcgctctcgaagttcctcttggcacttaagggactctgttgcttcttgtttctgtctaaatgactcacgcatcaactctgtctgtgtcactttcgcatgttcaagctgactgctagtttcacttatggcttctaggagtttttcaactgctgcttgtagtcgagagctaatgttcagcataagttcttcattttcagggtctatttcagttccagcaaaaccactcctcacaagtcgttgtgacagctctgttccttcctcagttacttttgaccacatgttaatgtcatttcttggcatatcacttccagaataagagggaatggattcatctgtaactcttgtatgttcctcatggacacatgactttacagatgcctctgcttctgacctccaaattaggctggcagatgactggcttttactagatctatctagaatcccaaggacatggcgaccaattgtttcttcaacagctgctgttgtctttacaacttctaagaggatcttcaaaagtctattattagctttctggagtgcatacactgtctttcttgtttgagttccatactgactgcgttccatactgatgatccaatggggaagccaaaatcttaggggccaaattcctccatgcaagctttcattagacaaaatctcaggaggcacatcttcaggttttctgtctaattccttttctttaaatgtttgttcttcaacttctccttggttttcatttccattctgtgtttgcgtactgctgttgcgcagctcacaacacagcttctctcttccagctaaagacagctgctttagtgcttccagctcctctaaaagcaccctctctctctctgaaaccaggttttcattatctatggaggatctctgggctaattgtctattaagtctcttaatctcttcttgtagctgttcctggtcttctcgctgtctctccatttgccgcatatgtgcttgccttaacaattccgttgcctgttgatgttcttggtattgtcgtacaagttcctgtctcatatcttccaactgttcttcattcaacattagttgtctagaagcatccatgcttgacactgaaatctcatcatgaatagactgtctaactataaatgttttatctttggagaacatttcttctgaaatagtcagcacacagtcctttgattctggtatatcatggggatcactatttgataataaaatttcctttccatgttctcctaactctttactaagtggtttaaattcttctttaaatttcacatccactgtctcaaaagtctgaaaaccaatttgatcctgtgataatttcatttcattaaaataatgttgttcttgctgacacacagcatgtgcttgctttgatgatgcagtattttcttttcccccagatattctagacagttcagtttgttgagcaaatgctatactcattgacacaataaccttagctacttcttcttctaattgttcttggtattgtttttcaagcaacttaacgatatttgtttcctctttcactccaaattcaccagaaaactctattgtaccatcaatattctttttcacacaacttccagggtacattgttctctgtgcatcagattctgtaattaccaccgaatcaacaggtaagcttggcggaaccgtggactcactaacagcttgaagcctcttctgtaaacagtggatctctgcctcatagttttgttcagtttctttcaactgttgctgcaaagaggatatgaggctttctaattcttgaacttgttcttcaagtttagttttttcaagatcttgcagagaagataacttgcttttatgattgacatcaatgtcttccaaattggtcatctgagaatggattgataaaaactctgtttcctcttttggaaggttttcttctccaaattcaagtttcataccatctgtctgctgtccccagatcttgcttagtcgtgtttgaagtaccaagagtttgttgtattcttctgttactttgttgagaagagtgtgcatattttcttgaaagtcttgaacttcatatctataatcttgtaattctggatcttcattttcagaaatgtaatcaccagaattctctttgtcttctgcatttacttcacattttaaagcaggagtataatattcaccaaggacactgcataaagtctgtaaaaaataagaacattcttcagacactgccttttgaagttttccaatgagcagatgtaaaggctttccttcatcacctgtttcttgtgttttcatagtctgtagttctaactggtgtattttctgaagttccttgatcttttcctcttgagcaaaaataagctcttctttaagactgcaaagagctttatctttttcattttccatatattcacgaacctgatccacatgagttgaataaaccagagagaggcaaatgcgttgggcttccatctgtagccttaaatcattctgttctgatttaagtacattgagttctttctgaagtttatcattttcacttggttgagttgctctaagtgatgattcctttgttacagatggtaagtgatccaaaatcaactgttcttgcttactttcttctccaacagtcatattttcaaaagaaactttatcttccaccattatttttgattcttcaccaaaacttttatttactttagaaactgatccttcagcacccctgcttgtcatggtcacaactccatctaataaagagcttacttgagtatcacatgactgtacattttctgccctgttgtggttaataatgatttctagctctctacatctcaatgaaacttgttctttctcttgctttaaagatttaacttcttcatttagaaaactaatctcaccatgtttctgtttcaattgttcagaaagatcagacagtctctgtgacagctctaatttctctcgcttggttacctcaagtttttccatgagttctgttgtatccttttcaacaacctcacccatttccaatgtttctgctacaaaagttttgtcttcatcaaagacagaacttttcattttcactgtagttggatttattctttgcaaatgaagctcttcattaagtgctttaagtttacttttatactctaattcctgtttatttttactgtcttctaaatcatcttttactttgagaaggcaagcatactcctcttgtaactcttgatagttaacttcaaagtttttttcagcaaatgaaaaagtgttcctttgcttttcaatctcttcatttagctgaatacattgttgtttgaggtcctcattttcctctataagtatttctatttctttttcccacacagagtctttggatttggacttaatggagtctaagaaaatcaatctttcttcttggctaacaggagtatgtattttcaacatgtcttcaagggttttcttttcatctttaagaatgctattctctgcttcaagttgtgcaaatttttcttgaagatcattctctttttccttcatctgtttttctaacaattctgttttaagttgtaattcttgaacttcttgttcaagtgtacccttttctttttcttcttgtctgagtatttcaatttctttttgaagttcattgatttgaagagtcatttcttctgactttgaatttacaagagactgctgtaaatcttttagctttgaaatttccaaaattaattgattctgcttagttatcaaattgtccttttcaaactgcatggtttctatcttttgactcatttcattctgtaaaccatctatctgctgtttatagtgaatgcctaaattatctttaagtttttcaatatttattcgatgttcaatttctaaatcttccttcagtttggaaagctcttcttcgtgactaaatagaagctgtgttctcagcctctctaattcagcttcttgtgattcagccattctgtctaacacagcattcttttctttttctaacatttcaagttttatcttgtaatttgtaacttctgcttcatgttttaattctagttcctttctggattcagatgcagaaacaatctcagctttcaaatcttccactgtactaagggacttatgtgcttcattaagtttactttcttgttcagctattgtctgtctagctctctgaatctgttcccttgaaaagctcaattcttcaacaaggtcttcaagctgtctctgtagagcacacttttcttctaaaattagtcctagttcttccttgagtttttccttttgagagttagtatcttgcaattttatattcagttcatttattgccacattcattaactttatctgatcttcattaactgtaatatttgaatatgaccttaaagcattctccatttctcccttatgccgtgttttcatttcctccatctgtgccatgtgttgtcttattaattcttgtttcatttgcactatctgctgcccatacatctcatccagctctgcccggagttgttctaactttctttgtgtttcttgttccattcgttgtactatatcagtttcgaactggctgtctttatgatttctcttctgaagttcttcgactgtccccattaactgttttatttcttcagaagactgtctttctttttgcttagaattagtcagctctaatttcatgttttttatttcttggttcttttgcacaatctgttcttgtaattctcctagtaatttatcagcagttgttaatttatcctttagctcaagagttttcttttcttcttctattatttttgtgtttaattcttcaatgattgtctccttttcctgtatttcttctttatttgagttttctacttttttatcttgttccatttcatatactttaattttctcttgcaagaaactaatttgcattgtgaagtcttctttctttttctgataatcttctaataagtggtcttgttcttcaagctgctgttgatgagtgaggatctgttgtttggcttgtagtaagtctgcagctgtgctactatgagtgctgtttctcagagtttcactagcctgtaattgctgaaattgaatctgtaatttttgactctgttctgtcaactctaaaaattctctcattgtctcatccttttctcttcttgcttgttgtaaattagcagtgagctgggttataatgccatctctttgtttaatggcagcttcaaattcttgtaactgctgcagtccttcagtcccataggtaaccctcatttcttccagctctctgtttagctcttcaatctcatgctgcttcccagccaactcactttccatcatctctagatgagtcggactgtcttgtgctccttgttcagaataagaatcatcaacaccaaattcttcttcccttaataaatttgtaggctttcctgttctcatcacaaaactgcaaccatttacctctgaactgcagtcatctgctgtggttgaaatttcactttccagagagttcagtactatctgtggtttcaggtctccactgggggtgttggactatactcttgatatggtttggctgagttcccccatccaaatctcatcttgaattgtagctcccataattcccatgtgtt

SEQ ID NO: 14130 - RNA, 16003 nt, Homo sapiens
  source 1..16003: mol_type = other RNA
gctgggattacaggcatgagccaccgcacctggccttccctgcttcctctctagaatccaattagggatgtttgttactactcatattgattaaaacagttaacaaacttttttctttttaaaatgtgagatcagtgaactctggttttaagataatctgaaacaaggtccttgggagtaataaaattggtcacattctgtaaagcacattctgtttaggaatcaacttatctcaaattgtaactcggggcctaactatatgagatggctgaaaaaataccacatcgtctgttttcactaggtgatgccaaaatattttgctttatgtatattacagttctttttaaaacactggaagactcatgttaaactctaattgtgaaggcagaatctctgctaatttttcagattaaaattctctttgaaaaaatacagtctgtattcatgaattgtaaaatatgtgcttcagtgagcagagttagggaatccaggaacttgggtggggaaaaattacatctttatttgcactaataatttctaactgcaatttagtatttatttcaattatgaatttgggcagcattttattagcagtatccatgattttgtcaatagaaatctcagatattttcatattacagatgttacagatttcttgaagtatctagttacgaccccgagataaggctagtctaatgtttagtgaatagttttagacttcttaacagatttcatttttaatcacagactaattaattattgagatgcataaacaagtgtgattgcagaggcctactatcataaggaggcgtggtggtcaaacaatggcactgaactcagcttgatcagatcatttgtccatctgtttttttctccactgtctcttagagcagaatagccttgaatggcaagccatgctagctgaaaaaggtttttacccacaacctgccccttcaactaactgctttagagtacgtttgctatttttagaattcctcttattggaacccagcttctaatgtggaaaatttaagtatagttggctccttttatttgtgggttctgtatcctctgattcaaccaactgcaggttcaaaatactaaaaataaaaccccacaataaaaaaatacagtattagcaactatttacataatgttcacattgtattaggtatcaaataatctggagatgatttgaagtacacaggaggatgtatgtagactatctgcaaatagcacattgttttataagagacttaagcattcgcggactgtaatatccaagggggatcctggaactaatcccccacacatgccgagggatgactgaaattagaaatgttcaagcatgtacaactttctaccatgcctgtttgtgttggtataaatcatggaacatcaaataataagacaaaatcctccaggtgtaagcatcaaatactagtcctcttgctgttttagtgagttgccatgttattgaggaggactccagatgagaaataacattgcgatctgtattatctctgtgagagcctcccagtctgaatttggcttggacaacagggatactgtttaattcggctgcaatgtgattaagatcttttgagttaatgatttcttcatctttttagtgggccatggatttgtgagaacacatctttggaaacaagtaacactaactgtaatatagtaaatactgattaatcatgaaataccaatatagcttttaaaaaacactatgtagatgtaaagttgatacaaagacacatggaaaactttcaacagtattaactctaagattaggacaactttctctgaatctctcactcctacatatttgacataagtaatgagatgctatgtaccaagaactatggctcagttaaaaatgaagaaggttcaaatacagtgtggtgaaaatggtgaagtcatttttatttcagtacttgacaaaataccccataaaattcaaaacttctaccattatacaaaaataggtctctacaagtgatattatctgtcttcatcaccagtagaatatattaggcaaaacatgtaacttcagtagccttataagaaaagtgcaggacacctcgagctacacattcagcagtattgtaatgcgtaaaagtttaatcttttcacccatttgataaatacacaaggtttataatttaatgttttaaattagcattccacaaatatacaggtaattcaataattattgtgcatgaatacatacacaatgcttatatatacaaattccagtttgttttcatgtgctggcaagggatttgtatacaatcataagctgtgttcatattggtcccattgaatattcacaatacaaaagcacaaaagaaccattgatttacaaaaggaaatctatttaaaatcacttcaattaatgatgtttcaaaggattatcttctcatgccagcatgaaattgagtagttgaacctatgagagaaaaacaggaaattcaactgatttcaaattacattgctacctgtatcagacccaccagagttcacacaaaggaaattattattattctccatttttttaaagccctttttttccttaaaatgtcctcttcatacttaaactgagtctctccccactacccccaaggtggagtgttactctgttgcccaggctggaattcagtggtgtgatcttggctcactgcaacccccgcctcctgggttcaagtgattctcctgcctcagcctcctgagtagctgggactatccacacatgccaccatgtccagcaaatttttgtatttttagtggagacggggtttcaccatgttggccaggctagtctcgaactggttggtcttgaactcctgacctagtgatccgcctgcctcggccgcccaaagtgctgggattacaggcatgagccaccgcgcccagcccatatacttaagctgacttttaagagattttgaatatatatgtaaaaatcaccatgactggctctatggcaaggtaggtgagactaatatttagagtttttttaaagtgctctcaaagttggatgttctatacctcatacatttttgaaaaatcttttggtcttcaaaatctgggtcttgtgaaatttggatgctcaaaacaaaacaagcctaggcaaaccaacaaactcagctatgataataaaagtttcctattactacaagatgcttgggtgtaaacaaatgatttcttgaaggaagagataaactactcaatgattcaaagtctctgaatcaggagtgaactgaagtgagatagggaaaagaggttttccttccatgaacagggaatccacctttattttaaagtatgacttgttttttgtttttgaacaaagaaaaaataatccttacaaagtattttaaatgggatagtttttttcgatgatacataaaagcacaatatagtagcagggataatggttacattaagtgcttaaagtaagtgcttcctccttaactccacccgatttgcatgccttaccactttcttttttttttttttttctttgagacagggtctcgctctgctgcccaggctggagtgctgcggcacggccttaccactttctgccatgcgctacttaggaatacgttctccagttaggctctgtagactcagagtaccttgcacactggtgctcattgtgcattttgtgtcatcagtccgctgaatgaacatagtaggaaatcatttttgggaggagtgggatctggggtgataaatcatattttcacttaaattatttaaagtcagtttctctgctggttacaagagtttaagctttggctaacttaataattagctcatgcactaaactggaagctttgattatcctaatgagtgtgaaagaatttcaaagaaaggggagctgtgggtctcgcactgtggtgctgccaagatgtggttaaactcagagcacctgactgtatagttccaagtcgtctttgcagtgcctctagccgagtgatataatctgttagggctctgtcaggatcgtaattctgaagctgagaacatgctaaagaaccaggattgaaatcagctggagtgcctgggtacctattctgaaatggtaaaggggacctaatatagtccagatctgatcttgagcgatacgtagtatgtcttggttctccatataactccagcccaccagaagaatgataaaatgagtcagtcttttctgcaccttgattcagtccaaagccatctctgttaatattgatggaaacagaacctgtgactcgatgccaccgtcgaaccaaaaatttcattctggaaattgcaatggatactctgacggccgaccgaaacctggtgaagccctttgggcgattggtgatcacctctagatccgtgaaagctggctgcccccccatccgggcaagcagggccaaggtggcatcttcacattcctggaacccacccagtaacagcagcaggtatttcttctggtaaatgagagcctttcgaaaactttctgccctcaagtatttaccataaattctctttaaagtgacatgttcagaatcagggctcagagtttgaagtaaagagtcatttcttagttcagctttcagtttgtatacttcagcctctgcccttttcaaagatttctggagagtcaatttttctctgttccatacttctttttcagaggcaatgatggcttcaatgttggcaccaccattcaatgaaaacctggaagaattatctctaccagctcctgtctgtcgataccacctgatctgctcttccagcttcataaccatgttccttaagtcattcttctcttcagtcagttgactgatatgccctgtcagctcagcattttgtctcagtagtctttcagtcaatgagccacaagaagtacttggggacaccaagctgggctcttcaccttgctggccagttaatttctgtagttgtaaaataatttcatcaatattttcctgaacccaaatgaaatcttcatcatctgctgtttcaaactgtagtctctcagaggctttctggggtagaacctgtagttttgaagctacacattgaagcttttgtctgatcatttctaattcatgattacagccggttcctcctccattcatttcaatcaatttagcgtagtttgattcttttgtttctccttctattttctgttgaagaacccaatttctagttctatcactggttaagctccacgtggttggctcattaaggttctgatacagaattcttctactttctcgtttttcttctcgttctagttcttgcttctggaattcctgcatgattccttgtagtcgctgtccttcaaggtctaacttataaacttgttgtcttttctcttccagctggcgctgaagatcttccactttggactggagctcatgcatttttttctgtccctcagtgttggcctcctgttctgtctgcagtgttttcctgtgaacctgcctatctttttccatttgctgtcgtgtttgcaaagaatccagtttatatttttcagtctcatttaacaattctactatgcgactgtgtttttcctctagctgtttctgcagctctttcagtaggtcctctgagggcaagggtggccgagactgtccagtaccatcactgctctgcagctgtgcgtgcaattcccgctccctatctagggtactactcatttcccgaattcgaactttctcagattcaagaagtacctgaagctctaagtttcgaccttgttcttctgacaactgggcatcatatagcattctctgtgattctattttttgctgggattcgttcagtagttgtttctgttgttccaaaagtagatttagctgaagattcctttgtttctgactctcaagtgaaaacttcagatcctcaagttcttctttatcccgttcttcactgcgtcccaacttggctttctctttctccaaagcccactggagctctcttgattttttctgttcacttgctaatgtgtcattaagcaaatgtacttcatctgtcttatctttaacttccaacctgaaagcctccaattcttttaggtgtttatgctgtgccttgagtgttgtttctagttccaatttagtttgtgcaagctcactcttcagttcagcaaccaccattttctcagaactcagctgctcctgcagttccgttgctctgtctttcatactgctgagctccacttgcatctccagcatttgagactgcttctgctgtatattatattccaagagttcttggcttggtttctcactctcttgttctcttttcagagtaattttcctaccattcatttgtgcatgcagtgcctgaatttcagataacaaactccttctatctgctttctggaggcattccatagctgcttgatattcaacaccctgttcttgtattctctgttccaaacagtttagtaaaccaactgcatctgtagtacctagagctgtcagctccgtccgaaatgctgctagtaaaacactacgctcttctaagaaaacttgttgaagggcaagcagtagttcacctcgccagtctgagaagctctcatgagattgagaactatcataaacctcggcttctctttgcagttgcatctttgtaattaaatcctttagagatgagattgtattgatgtaagcttttctctcttctagccaaggttctgaaacctgctgaatagaatggtcctctccatcactatagggagactcagtgagagaaagcacctgcatgccttcattatggacagctctcagtaatccctttattttctttggaaaggaatctgttgcactttcactttcttctcctcggccttctgatgctatgtcaaatccctgactgtgtgtaagataaattccctgaccccagtctgatccagaatcactggagcatatttctctagtctggtaagcatcagaatgtgctagctcaggaattgaggatccctctttacttctcagacactgtatcactgccttcaaggtaccacattcctctttcagtaactgaacggcaacatagtgttccctctttaaggtttcagtttctgaaatatgtctggattccatgtccaaaatttcagcagcatgtagttcttgcatcttctcaattttttcagtaaactgactgattatttcagtaacttcttctgaggaacattcactctgtaaattaatttgtattcctgcatttttaacaagaatttgtggagtctgattgctgctactgatcttcagagtcccatctgtctgggatgcaatgctcttactcagttttataggaagtggctcaaacatgcaggcctttttgctttcttgtacctcagtctcatcttctttttctaaaatggacaatttctcttttgcctctgcgaggtgatccctaacttggcttaagtctttctgaagagatgtcatatttgtttcttttaccaaaagctcttcttgaagtttttcagccttttctttataactggcaagttctgctttggtagccactgattcagctctaagagcctcgagttcattaaaaaatccactttcttcattgctatgaaatagctcagtagttgtcttgagaacttcaacatcttgagggcttcttttcttttctttctctctctgttttttctcattgccctccaatagcttctgtagttctagcagcttcttttctttttctaaaacatttttttctgcaatttctacttgttctttttctaaaatcaaactagtatgcatttcaacaacctggctttctaattctgatattctcaaggttaatgctgatatatctgaccccaactcatcttctcttagttgatttaaattctgaatatttgttctttcaggttctgatgaaattgtttgattatcttgacagaattttgcatattcctgaactgcctcaagttggatttgactgacaagagcagcagccactttttcttcaactattttctgtaggtttacaatcttcttttgaagcatttctgtttcaaactggccttgttcttgcatgtcttttatttgtttataacactgggtaagttctaagtcctttgcactaacagtgctctcaagttgtagcaaccttgtttccaaattaattatggaacctttgccattttcttcaaaagatttgaagtatgtctgattttctagggatttaagagcatcctctgtaaggactacttctagttcaggtttgtctttgctcagatgatctatagccacgttaacactattctctggtatgctttgaatcttttccacactttcacgttctctctttaagctgaataattcctgtgttagctgattcattttaaaattggtttctttaagtacatttttcatgaaggtcatttcttcattagcggtttctacttgctgttccaaggccagcttttcagctataaccacatccaattgatgttttaaactgtctgcttcttctgagagggaatgagcattcattgatgtcttctgtccaatatttgccaattcctgttgaagtttttcaatcacttcattgagctgctctatttcttcttctctatttctcttcacacattcttgatcactcatcaaacattctatttgggtttcaagatcccttatcagttcatttttttcttcaataaccttgttatctgttgtaattttaagttgctgctggagtttcgtaacttgttcatttaattggtcaatttctacctctttttcctgtattatttgagcaaatttcccaaatagcacatgttggtcttgagtagacatggcatcagattcctttatggcaagtcccagtttctccatgtcatccttaaataatttgttttcctgttcaagttcttgtaggcgggtagtagattcctttttctgtatttctaattgcatatgtaattgttgaacttcttcattcttattttccagttcttctctaaactgttctaattgctcttctaagtttgtaatctctttttcctttctgtctatggcatctcgttcagcctgcaattgtacttctagggacaattctggtttagcttctacagctccaaagtgttttcggtcctctaccttttgaaaagtatctgcactcacaagaagcgcctgctccagttctcttactctgaactccagtttctctatttcttcattcctttcttgtatatccctttgaagctgctctttagagagcaaaagctcactgcatttgtctgttttttctttcagatgatttgctaactgttcaacctctctagtttgatgttcactgataggctggaatcgaggaacaaccttaagttgctgttctagtttctgtatttcctgttggaatacatctctctcatgttctctgtcaatggcttgctcatctaaaaattttctcattttttctaactgcttttccaatgcttggttttgctgtcttaaatccattagttcagtatttttttcttgttccagctctataaacctactgacttgttcttccacatctatttctagagctttcacttgtttttgaaggtcatcacgtactttttcagcttgacattgtacttctagtttttccttcattaatttttctgtctcctgtagtaattctgctcctggtgctgcatcgactgcagcatctactagtcgttgttcaactgggcctgcctctgctttcatagcttccttttgtctggacagtaattctctttcttcttggatctgctgttgctctgcctccaattcttgcaacctgttacttgcacataacaactcctgctcaagacgatctattatatcagttttttcctgaatttgcctttcaaaaagagttttttcatctgcatagccatcaatgacgccctcagccttactgagctccacagctagctgttctctggccctggactcctcatgaaggcgctctcgaagttcctcttggcacttaagggactctgttgcttcttgtttctgtctaaatgactcacgcatcaactctgtctgtgtcactttcgcatgttcaagctgactgctagtttcacttatggcttctaggagtttttcaactgctgcttgtagtcgagagctaatgttcagcataagttcttcattttcagggtctatttcagttccagcaaaaccactcctcacaagtcgttgtgacagctctgttccttcctcagttacttttgaccacatgttaatgtcatttcttggcatatcacttccagaataagagggaatggattcatctgtaactcttgtatgttcctcatggacacatgactttacagatgcctctgcttctgacctccaaattaggctggcagatgactggcttttactagatctatctagaatcccaaggacatggcgaccaattgtttcttcaacagctgctgttgtctttacaacttctaagaggatcttcaaaagtctattattagctttctggagtgcatacactgtctttcttgtttgagttccatactgactgcgttccatactgatgatccaatggggaagccaaaatcttaggggccaaattcctccatgcaagctttcattagacaaaatctcaggaggcacatcttcaggttttctgtctaattccttttctttaaatgtttgttcttcaacttctccttggttttcatttccattctgtgtttgcgtactgctgttgcgcagctcacaacacagcttctctcttccagctaaagacagctgctttagtgcttccagctcctctaaaagcaccctctctctctctgaaaccaggttttcattatctatggaggatctctgggctaattgtctattaagtctcttaatctcttcttgtagctgttcctggtcttctcgctgtctctccatttgccgcatatgtgcttgccttaacaattccgttgcctgttgatgttcttggtattgtcgtacaagttcctgtctcatatcttccaactgttcttcattcaacattagttgtctagaagcatccatgcttgacactgaaatctcatcatgaatagactgtctaactataaatgttttatctttggagaacatttcttctgaaatagtcagcacacagtcctttgattctggtatatcatggggatcactatttgataataaaatttcctttccatgttctcctaactctttactaagtggtttaaattcttctttaaatttcacatccactgtctcaaaagtctgaaaaccaatttgatcctgtgataatttcatttcattaaaataatgttgttcttgctgacacacagcatgtgcttgctttgatgatgcagtattttcttttcccccagatattctagacagttcagtttgttgagcaaatgctatactcattgacacaataaccttagctacttcttcttctaattgttcttggtattgtttttcaagcaacttaacgatatttgtttcctctttcactccaaattcaccagaaaactctattgtaccatcaatattctttttcacacaacttccagggtacattgttctctgtgcatcagattctgtaattaccaccgaatcaacaggtaagcttggcggaaccgtggactcactaacagcttgaagcctcttctgtaaacagtggatctctgcctcatagttttgttcagtttctttcaactgttgctgcaaagaggatatgaggctttctaattcttgaacttgttcttcaagtttagttttttcaagatcttgcagagaagataacttgcttttatgattgacatcaatgtcttccaaattggtcatctgagaatggattgataaaaactctgtttcctcttttggaaggttttcttctccaaattcaagtttcataccatctgtctgctgtccccagatcttgcttagtcgtgtttgaagtaccaagagtttgttgtattcttctgttactttgttgagaagagtgtgcatattttcttgaaagtcttgaacttcatatctataatcttgtaattctggatcttcattttcagaaatgtaatcaccagaattctctttgtcttctgcatttacttcacattttaaagcaggagtataatattcaccaaggacactgcataaagtctgtaaaaaataagaacattcttcagacactgccttttgaagttttccaatgagcagatgtaaaggctttccttcatcacctgtttcttgtgttttcatagtctgtagttctaactggtgtattttctgaagttccttgatcttttcctcttgagcaaaaataagctcttctttaagactgcaaagagctttatctttttcattttccatatattcacgaacctgatccacatgagttgaataaaccagagagaggcaaatgcgttgggcttccatctgtagccttaaatcattctgttctgatttaagtacattgagttctttctgaagtttatcattttcacttggttgagttgctctaagtgatgattcctttgttacagatggtaagtgatccaaaatcaactgttcttgcttactttcttctccaacagtcatattttcaaaagaaactttatcttccaccattatttttgattcttcaccaaaacttttatttactttagaaactgatccttcagcacccctgcttgtcatggtcacaactccatctaataaagagcttacttgagtatcacatgactgtacattttctgccctgttgtggttaataatgatttctagctctctacatctcaatgaaacttgttctttctcttgctttaaagatttaacttcttcatttagaaaactaatctcaccatgtttctgtttcaattgttcagaaagatcagacagtctctgtgacagctctaatttctctcgcttggttacctcaagtttttccatgagttctgttgtatccttttcaacaacctcacccatttccaatgtttctgctacaaaagttttgtcttcatcaaagacagaacttttcattttcactgtagttggatttattctttgcaaatgaagctcttcattaagtgctttaagtttacttttatactctaattcctgtttatttttactgtcttctaaatcatcttttactttgagaaggcaagcatactcctcttgtaactcttgatagttaacttcaaagtttttttcagcaaatgaaaaagtgttcctttgcttttcaatctcttcatttagctgaatacattgttgtttgaggtcctcattttcctctataagtatttctatttctttttcccacacagagtctttggatttggacttaatggagtctaagaaaatcaatctttcttcttggctaacaggagtatgtattttcaacatgtcttcaagggttttcttttcatctttaagaatgctattctctgcttcaagttgtgcaaatttttcttgaagatcattctctttttccttcatctgtttttctaacaattctgttttaagttgtaattcttgaacttcttgttcaagtgtacccttttctttttcttcttgtctgagtatttcaatttctttttgaagttcattgatttgaagagtcatttcttctgactttgaatttacaagagactgctgtaaatcttttagctttgaaatttccaaaattaattgattctgcttagttatcaaattgtccttttcaaactgcatggtttctatcttttgactcatttcattctgtaaaccatctatctgctgtttatagtgaatgcctaaattatctttaagtttttcaatatttattcgatgttcaatttctaaatcttccttcagtttggaaagctcttcttcgtgactaaatagaagctgtgttctcagcctctctaattcagcttcttgtgattcagccattctgtctaacacagcattcttttctttttctaacatttcaagttttatcttgtaatttgtaacttctgcttcatgttttaattctagttcctttctggattcagatgcagaaacaatctcagctttcaaatcttccactgtactaagggacttatgtgcttcattaagtttactttcttgttcagctattgtctgtctagctctctgaatctgttcccttgaaaagctcaattcttcaacaaggtcttcaagctgtctctgtagagcacacttttcttctaaaattagtcctagttcttccttgagtttttccttttgagagttagtatcttgcaattttatattcagttcatttattgccacattcattaactttatctgatcttcattaactgtaatatttgaatatgaccttaaagcattctccatttctcccttatgccgtgttttcatttcctccatctgtgccatgtgttgtcttattaattcttgtttcatttgcactatctgctgcccatacatctcatccagctctgcccggagttgttctaactttctttgtgtttcttgttccattcgttgtactatatcagtttcgaactggctgtctttatgatttctcttctgaagttcttcgactgtccccattaactgttttatttcttcagaagactgtctttctttttgcttagaattagtcagctctaatttcatgttttttatttcttggttcttttgcacaatctgttcttgtaattctcctagtaatttatcagcagttgttaatttatcctttagctcaagagttttcttttcttcttctattatttttgtgtttaattcttcaatgattgtctccttttcctgtatttcttctttatttgagttttctacttttttatcttgttccatttcatatactttaattttctcttgcaagaaactaatttgcattgtgaagtcttctttctttttctgataatcttctaataagtggtcttgttcttcaagctgctgttgatgagtgaggatctgttgtttggcttgtagtaagtctgcagctgtgctactatgagtgctgtttctcagagtttcactagcctgtaattgctgaaattgaatctgtaatttttgactctgttctgtcaactctaaaaattctctcattgtctcatccttttctcttcttgcttgttgtaaattagcagtgagctgggttataatgccatctctttgtttaatggcagcttcaaattcttgtaactgctgcagtccttcagtcccataggtaaccctcatttcttccagctctctgtttagctcttcaatctcatgctgcttcccagccaactcactttccatcatctctagatgagtcggactgtcttgtgctccttgttcagaataagaatcatcaacaccaaattcttcttcccttaataaatttgtaggctttcctgttctcatcacaaaactgcaaccatttacctctgaactgcagtcatctgctgtggttgaaatttcactttccagttccacagagaagccctgctcatgactggttatttctccactatgtagagttctcattattgtagattcaggaatcacagttgattctactctctgagaactatttatgtacatttcattacactgtgattgatcaatattcaaatcatggtgtgctgacacatcatgtttactgcttgacgtttttctcttttttttctgcttcttggaaggactctgcccatccgactgagcttttctttgtcgaaactgggcaagcttggctttgccggcctccagcttcttctgtctctcctcgtcctccatggcctctgcaaggaaggcaggggaaaacaggggttgaggggtggttggggatagaaaggaaaggtcgatttggacggaggtgggacggcaagctccacggcctagagagccgattcggtccggcgctcccccgcccgaagtggaagcagtctccgcgctcactggcggatcgtcctcagccgcacgggaagcgccgtcaccgccgccgccgccgccatcttcgtctccacgta

SEQ ID NO: 14131 - RNA, 15662 nt, Homo sapiens
  source 1..15662: mol_type = other RNA
gctgggattacaggcatgagccaccgcacctggccttccctgcttcctctctagaatccaattagggatgtttgttactactcatattgattaaaacagttaacaaacttttttctttttaaaatgtgagatcagtgaactctggttttaagataatctgaaacaaggtccttgggagtaataaaattggtcacattctgtaaagcacattctgtttaggaatcaacttatctcaaattgtaactcggggcctaactatatgagatggctgaaaaaataccacatcgtctgttttcactaggtgatgccaaaatattttgctttatgtatattacagttctttttaaaacactggaagactcatgttaaactctaattgtgaaggcagaatctctgctaatttttcagattaaaattctctttgaaaaaatacagtctgtattcatgaattgtaaaatatgtgcttcagtgagcagagttagggaatccaggaacttgggtggggaaaaattacatctttatttgcactaataatttctaactgcaatttagtatttatttcaattatgaatttgggcagcattttattagcagtatccatgattttgtcaatagaaatctcagatattttcatattacagatgttacagatttcttgaagtatctagttacgaccccgagataaggctagtctaatgtttagtgaatagttttagacttcttaacagatttcatttttaatcacagactaattaattattgagatgcataaacaagtgtgattgcagaggcctactatcataaggaggcgtggtggtcaaacaatggcactgaactcagcttgatcagatcatttgtccatctgtttttttctccactgtctcttagagcagaatagccttgaatggcaagccatgctagctgaaaaaggtttttacccacaacctgccccttcaactaactgctttagagtacgtttgctatttttagaattcctcttattggaacccagcttctaatgtggaaaatttaagtatagttggctccttttatttgtgggttctgtatcctctgattcaaccaactgcaggttcaaaatactaaaaataaaaccccacaataaaaaaatacagtattagcaactatttacataatgttcacattgtattaggtatcaaataatctggagatgatttgaagtacacaggaggatgtatgtagactatctgcaaatagcacattgttttataagagacttaagcattcgcggactgtaatatccaagggggatcctggaactaatcccccacacatgccgagggatgactgaaattagaaatgttcaagcatgtacaactttctaccatgcctgtttgtgttggtataaatcatggaacatcaaataataagacaaaatcctccaggtgtaagcatcaaatactagtcctcttgctgttttagtgagttgccatgttattgaggaggactccagatgagaaataacattgcgatctgtattatctctgtgagagcctcccagtctgaatttggcttggacaacagggatactgtttaattcggctgcaatgtgattaagatcttttgagttaatgatttcttcatctttttagtgggccatggatttgtgagaacacatctttggaaacaagtaacactaactgtaatatagtaaatactgattaatcatgaaataccaatatagcttttaaaaaacactatgtagatgtaaagttgatacaaagacacatggaaaactttcaacagtattaactctaagattaggacaactttctctgaatctctcactcctacatatttgacataagtaatgagatgctatgtaccaagaactatggctcagttaaaaatgaagaaggttcaaatacagtgtggtgaaaatggtgaagtcatttttatttcagtacttgacaaaataccccataaaattcaaaacttctaccattatacaaaaataggtctctacaagtgatattatctgtcttcatcaccagtagaatatattaggcaaaacatgtaacttcagtagccttataagaaaagtgcaggacacctcgagctacacattcagcagtattgtaatgcgtaaaagtttaatcttttcacccatttgataaatacacaaggtttataatttaatgttttaaattagcattccacaaatatacaggtaattcaataattattgtgcatgaatacatacacaatgcttatatatacaaattccagtttgttttcatgtgctggcaagggatttgtatacaatcataagctgtgttcatattggtcccattgaatattcacaatacaaaagcacaaaagaaccattgatttacaaaaggaaatctatttaaaatcacttcaattaatgatgtttcaaaggattatcttctcatgccagcatgaaattgagtagttgaacctatgagagaaaaacaggaaattcaactgatttcaaattacattgctacctgtatcagacccaccagagttcacacaaaggaaattattattattctccatttttttaaagccctttttttccttaaaatgtcctcttcatacttaaactgagtctctccccactacccccaaggtggagtgttactctgttgcccaggctggaattcagtggtgtgatcttggctcactgcaacccccgcctcctgggttcaagtgattctcctgcctcagcctcctgagtagctgggactatccacacatgccaccatgtccagcaaatttttgtatttttagtggagacggggtttcaccatgttggccaggctagtctcgaactggttggtcttgaactcctgacctagtgatccgcctgcctcggccgcccaaagtgctgggattacaggcatgagccaccgcgcccagcccatatacttaagctgacttttaagagattttgaatatatatgtaaaaatcaccatgactggctctatggcaaggtaggtgagactaatatttagagtttttttaaagtgctctcaaagttggatgttctatacctcatacatttttgaaaaatcttttggtcttcaaaatctgggtcttgtgaaatttggatgctcaaaacaaaacaagcctaggcaaaccaacaaactcagctatgataataaaagtttcctattactacaagatgcttgggtgtaaacaaatgatttcttgaaggaagagataaactactcaatgattcaaagtctctgaatcaggagtgaactgaagtgagatagggaaaagaggttttccttccatgaacagggaatccacctttattttaaagtatgacttgttttttgtttttgaacaaagaaaaaataatccttacaaagtattttaaatgggatagtttttttcgatgatacataaaagcacaatatagtagcagggataatggttacattaagtgcttaaagtaagtgcttcctccttaactccacccgatttgcatgccttaccactttcttttttttttttttttctttgagacagggtctcgctctgctgcccaggctggagtgctgcggcacggccttaccactttctgccatgcgctacttaggaatacgttctccagttaggctctgtagactcagagtaccttgcacactggtgctcattgtgcattttgtgtcatcagtccgctgaatgaacatagtaggaaatcatttttgggaggagtgggatctggggtgataaatcatattttcacttaaattatttaaagtcagtttctctgctggttacaagagtttaagctttggctaacttaataattagctcatgcactaaactggaagctttgattatcctaatgagtgtgaaagaatttcaaagaaaggggagctgtgggtctcgcactgtggtgctgccaagatgtggttaaactcagagcacctgactgtatagttccaagtcgtctttgcagtgcctctagccgagtgatataatctgttagggctctgtcaggatcgtaattctgaagctgagaacatgctaaagaaccaggattgaaatcagctggagtgcctgggtacctattctgaaatggtaaaggggacctaatatagtccagatctgatcttgagcgatacgtagtatgtcttggttctccatataactccagcccaccagaagaatgataaaatgagtcagtcttttctgcaccttgattcagtccaaagccatctctgttaatattgatggaaacagaacctgtgactcgatgccaccgtcgaaccaaaaatttcattctggaaattgcaatggatactctgacggccgaccgaaacctggtgaagccctttgggcgattggtgatcacctctagatccgtgaaagctggctgcccccccatccgggcaagcagggccaaggtggcatcttcacattcctggaacccacccagtaacagcagcaggtatttcttctggtaaatgagagcctttcgaaaactttctgccctcaagtatttaccataaattctctttaaagtgacatgttcagaatcagggctcagagtttgaagtaaagagtcatttcttagttcagctttcagtttgtatacttcagcctctgcccttttcaaagatttctggagagtcaatttttctctgttccatacttctttttcagaggcaatgatggcttcaatgttggcaccaccattcaatgaaaacctggaagaattatctctaccagctcctgtctgtcgataccacctgatctgctcttccagcttcataaccatgttccttaagtcattcttctcttcagtcagttgactgatatgccctgtcagctcagcattttgtctcagtagtctttcagtcaatgagccacaagaagtacttggggacaccaagctgggctcttcaccttgctggccagttaatttctgtagttgtaaaataatttcatcaatattttcctgaacccaaatgaaatcttcatcatctgctgtttcaaactgtagtctctcagaggctttctggggtagaacctgtagttttgaagctacacattgaagcttttgtctgatcatttctaattcatgattacagccggttcctcctccattcatttcaatcaatttagcgtagtttgattcttttgtttctccttctattttctgttgaagaacccaatttctagttctatcactggttaagctccacgtggttggctcattaaggttctgatacagaattcttctactttctcgtttttcttctcgttctagttcttgcttctggaattcctgcatgattccttgtagtcgctgtccttcaaggtctaacttataaacttgttgtcttttctcttccagctggcgctgaagatcttccactttggactggagctcatgcatttttttctgtccctcagtgttggcctcctgttctgtctgcagtgttttcctgtgaacctgcctatctttttccatttgctgtcgtgtttgcaaagaatccagtttatatttttcagtctcatttaacaattctactatgcgactgtgtttttcctctagctgtttctgcagctctttcagtaggtcctctgagggcaagggtggccgagactgtccagtaccatcactgctctgcagctgtgcgtgcaattcccgctccctatctagggtactactcatttcccgaattcgaactttctcagattcaagaagtacctgaagctctaagtttcgaccttgttcttctgacaactgggcatcatatagcattctctgtgattctattttttgctgggattcgttcagtagttgtttctgttgttccaaaagtagatttagctgaagattcctttgtttctgactctcaagtgaaaacttcagatcctcaagttcttctttatcccgttcttcactgcgtcccaacttggctttctctttctccaaagcccactggagctctcttgattttttctgttcacttgctaatgtgtcattaagcaaatgtacttcatctgtcttatctttaacttccaacctgaaagcctccaattcttttaggtgtttatgctgtgccttgagtgttgtttctagttccaatttagtttgtgcaagctcactcttcagttcagcaaccaccattttctcagaactcagctgctcctgcagttccgttgctctgtctttcatactgctgagctccacttgcatctccagcatttgagactgcttctgctgtatattatattccaagagttcttggcttggtttctcactctcttgttctcttttcagagtaattttcctaccattcatttgtgcatgcagtgcctgaatttcagataacaaactccttctatctgctttctggaggcattccatagctgcttgatattcaacaccctgttcttgtattctctgttccaaacagtttagtaaaccaactgcatctgtagtacctagagctgtcagctccgtccgaaatgctgctagtaaaacactacgctcttctaagaaaacttgttgaagggcaagcagtagttcacctcgccagtctgagaagctctcatgagattgagaactatcataaacctcggcttctctttgcagttgcatctttgtaattaaatcctttagagatgagattgtattgatgtaagcttttctctcttctagccaaggttctgaaacctgctgaatagaatggtcctctccatcactatagggagactcagtgagagaaagcacctgcatgccttcattatggacagctctcagtaatccctttattttctttggaaaggaatctgttgcactttcactttcttctcctcggccttctgatgctatgtcaaatccctgactgtgtgtaagataaattccctgaccccagtctgatccagaatcactggagcatatttctctagtctggtaagcatcagaatgtgctagctcaggaattgaggatccctctttacttctcagacactgtatcactgccttcaaggtaccacattcctctttcagtaactgaacggcaacatagtgttccctctttaaggtttcagtttctgaaatatgtctggattccatgtccaaaatttcagcagcatgtagttcttgcatcttctcaattttttcagtaaactgactgattatttcagtaacttcttctgaggaacattcactctgtaaattaatttgtattcctgcatttttaacaagaatttgtggagtctgattgctgctactgatcttcagagtcccatctgtctgggatgcaatgctcttactcagttttataggaagtggctcaaacatgcaggcctttttgctttcttgtacctcagtctcatcttctttttctaaaatggacaatttctcttttgcctctgcgaggtgatccctaacttggcttaagtctttctgaagagatgtcatatttgtttcttttaccaaaagctcttcttgaagtttttcagccttttctttataactggcaagttctgctttggtagccactgattcagctctaagagcctcgagttcattaaaaaatccactttcttcattgctatgaaatagctcagtagttgtcttgagaacttcaacatcttgagggcttcttttcttttctttctctctctgttttttctcattgccctccaatagcttctgtagttctagcagcttcttttctttttctaaaacatttttttctgcaatttctacttgttctttttctaaaatcaaactagtatgcatttcaacaacctggctttctaattctgatattctcaaggttaatgctgatatatctgaccccaactcatcttctcttagttgatttaaattctgaatatttgttctttcaggttctgatgaaattgtttgattatcttgacagaattttgcatattcctgaactgcctcaagttggatttgactgacaagagcagcagccactttttcttcaactattttctgtaggtttacaatcttcttttgaagcatttctgtttcaaactggccttgttcttgcatgtcttttatttgtttataacactgggtaagttctaagtcctttgcactaacagtgctctcaagttgtagcaaccttgtttccaaattaattatggaacctttgccattttcttcaaaagatttgaagtatgtctgattttctagggatttaagagcatcctctgtaaggactacttctagttcaggtttgtctttgctcagatgatctatagccacgttaacactattctctggtatgctttgaatcttttccacactttcacgttctctctttaagctgaataattcctgtgttagctgattcattttaaaattggtttctttaagtacatttttcatgaaggtcatttcttcattagcggtttctacttgctgttccaaggccagcttttcagctataaccacatccaattgatgttttaaactgtctgcttcttctgagagggaatgagcattcattgatgtcttctgtccaatatttgccaattcctgttgaagtttttcaatcacttcattgagctgctctatttcttcttctctatttctcttcacacattcttgatcactcatcaaacattctatttgggtttcaagatcccttatcagttcatttttttcttcaataaccttgttatctgttgtaattttaagttgctgctggagtttcgtaacttgttcatttaattggtcaatttctacctctttttcctgtattatttgagcaaatttcccaaatagcacatgttggtcttgagtagacatggcatcagattcctttatggcaagtcccagtttctccatgtcatccttaaataatttgttttcctgttcaagttcttgtaggcgggtagtagattcctttttctgtatttctaattgcatatgtaattgttgaacttcttcattcttattttccagttcttctctaaactgttctaattgctcttctaagtttgtaatctctttttcctttctgtctatggcatctcgttcagcctgcaattgtacttctagggacaattctggtttagcttctacagctccaaagtgttttcggtcctctaccttttgaaaagtatctgcactcacaagaagcgcctgctccagttctcttactctgaactccagtttctctatttcttcattcctttcttgtatatccctttgaagctgctctttagagagcaaaagctcactgcatttgtctgttttttctttcagatgatttgctaactgttcaacctctctagtttgatgttcactgataggctggaatcgaggaacaaccttaagttgctgttctagtttctgtatttcctgttggaatacatctctctcatgttctctgtcaatggcttgctcatctaaaaattttctcattttttctaactgcttttccaatgcttggttttgctgtcttaaatccattagttcagtatttttttcttgttccagctctataaacctactgacttgttcttccacatctatttctagagctttcacttgtttttgaaggtcatcacgtactttttcagcttgacattgtacttctagtttttccttcattaatttttctgtctcctgtagtaattctgctcctggtgctgcatcgactgcagcatctactagtcgttgttcaactgggcctgcctctgctttcatagcttccttttgtctggacagtaattctctttcttcttggatctgctgttgctctgcctccaattcttgcaacctgttacttgcacataacaactcctgctcaagacgatctattatatcagttttttcctgaatttgcctttcaaaaagagttttttcatctgcatagccatcaatgacgccctcagccttactgagctccacagctagctgttctctggccctggactcctcatgaaggcgctctcgaagttcctcttggcacttaagggactctgttgcttcttgtttctgtctaaatgactcacgcatcaactctgtctgtgtcactttcgcatgttcaagctgactgctagtttcacttatggcttctaggagtttttcaactgctgcttgtagtcgagagctaatgttcagcataagttcttcattttcagggtctatttcagttccagcaaaaccactcctcacaagtcgttgtgacagctctgttccttcctcagttacttttgaccacatgttaatgtcatttcttggcatatcacttccagaataagagggaatggattcatctgtaactcttgtatgttcctcatggacacatgactttacagatgcctctgcttctgacctccaaattaggctggcagatgactggcttttactagatctatctagaatcccaaggacatggcgaccaattgtttcttcaacagctgctgttgtctttacaacttctaagaggatcttcaaaagtctattattagctttctggagtgcatacactgtctttcttgtttgagttccatactgactgcgttccatactgatgatccaatggggaagccaaaatcttaggggccaaattcctccatgcaagctttcattagacaaaatctcaggaggcacatcttcaggttttctgtctaattccttttctttaaatgtttgttcttcaacttctccttggttttcatttccattctgtgtttgcgtactgctgttgcgcagctcacaacacagcttctctcttccagctaaagacagctgctttagtgcttccagctcctctaaaagcaccctctctctctctgaaaccaggttttcattatctatggaggatctctgggctaattgtctattaagtctcttaatctcttcttgtagctgttcctggtcttctcgctgtctctccatttgccgcatatgtgcttgccttaacaattccgttgcctgttgatgttcttggtattgtcgtacaagttcctgtctcatatcttccaactgttcttcattcaacattagttgtctagaagcatccatgcttgacactgaaatctcatcatgaatagactgtctaactataaatgttttatctttggagaacatttcttctgaaatagtcagcacacagtcctttgattctggtatatcatggggatcactatttgataataaaatttcctttccatgttctcctaactctttactaagtggtttaaattcttctttaaatttcacatccactgtctcaaaagtctgaaaaccaatttgatcctgtgataatttcatttcattaaaataatgttgttcttgctgacacacagcatgtgcttgctttgatgatgcagtattttcttttcccccagatattctagacagttcagtttgttgagcaaatgctatactcattgacacaataaccttagctacttcttcttctaattgttcttggtattgtttttcaagcaacttaacgatatttgtttcctctttcactccaaattcaccagaaaactctattgtaccatcaatattctttttcacacaacttccagggtacattgttctctgtgcatcagattctgtaattaccaccgaatcaacaggtaagcttggcggaaccgtggactcactaacagcttgaagcctcttctgtaaacagtggatctctgcctcatagttttgttcagtttctttcaactgttgctgcaaagaggatatgaggctttctaattcttgaacttgttcttcaagtttagttttttcaagatcttgcagagaagataacttgcttttatgattgacatcaatgtcttccaaattggtcatctgagaatggattgataaaaactctgtttcctcttttggaaggttttcttctccaaattcaagtttcataccatctgtctgctgtccccagatcttgcttagtcgtgtttgaagtaccaagagtttgttgtattcttctgttactttgttgagaagagtgtgcatattttcttgaaagtcttgaacttcatatctataatcttgtaattctggatcttcattttcagaaatgtaatcaccagaattctctttgtcttctgcatttacttcacattttaaagcaggagtataatattcaccaaggacactgcataaagtctgtaaaaaataagaacattcttcagacactgccttttgaagttttccaatgagcagatgtaaaggctttccttcatcacctgtttcttgtgttttcatagtctgtagttctaactggtgtattttctgaagttccttgatcttttcctcttgagcaaaaataagctcttctttaagactgcaaagagctttatctttttcattttccatatattcacgaacctgatccacatgagttgaataaaccagagagaggcaaatgcgttgggcttccatctgtagccttaaatcattctgttctgatttaagtacattgagttctttctgaagtttatcattttcacttggttgagttgctctaagtgatgattcctttgttacagatggtaagtgatccaaaatcaactgttcttgcttactttcttctccaacagtcatattttcaaaagaaactttatcttccaccattatttttgattcttcaccaaaacttttatttactttagaaactgatccttcagcacccctgcttgtcatggtcacaactccatctaataaagagcttacttgagtatcacatgactgtacattttctgccctgttgtggttaataatgatttctagctctctacatctcaatgaaacttgttctttctcttgctttaaagatttaacttcttcatttagaaaactaatctcaccatgtttctgtttcaattgttcagaaagatcagacagtctctgtgacagctctaatttctctcgcttggttacctcaagtttttccatgagttctgttgtatccttttcaacaacctcacccatttccaatgtttctgctacaaaagttttgtcttcatcaaagacagaacttttcattttcactgtagttggatttattctttgcaaatgaagctcttcattaagtgctttaagtttacttttatactctaattcctgtttatttttactgtcttctaaatcatcttttactttgagaaggcaagcatactcctcttgtaactcttgatagttaacttcaaagtttttttcagcaaatgaaaaagtgttcctttgcttttcaatctcttcatttagctgaatacattgttgtttgaggtcctcattttcctctataagtatttctatttctttttcccacacagagtctttggatttggacttaatggagtctaagaaaatcaatctttcttcttggctaacaggagtatgtattttcaacatgtcttcaagggttttcttttcatctttaagaatgctattctctgcttcaagttgtgcaaatttttcttgaagatcattctctttttccttcatctgtttttctaacaattctgttttaagttgtaattcttgaacttcttgttcaagtgtacccttttctttttcttcttgtctgagtatttcaatttctttttgaagttcattgatttgaagagtcatttcttctgactttgaatttacaagagactgctgtaaatcttttagctttgaaatttccaaaattaattgattctgcttagttatcaaattgtccttttcaaactgcatggtttctatcttttgactcatttcattctgtaaaccatctatctgctgtttatagtgaatgcctaaattatctttaagtttttcaatatttattcgatgttcaatttctaaatcttccttcagtttggaaagctcttcttcgtgactaaatagaagctgtgttctcagcctctctaattcagcttcttgtgattcagccattctgtctaacacagcattcttttctttttctaacatttcaagttttatcttgtaatttgtaacttctgcttcatgttttaattctagttcctttctggattcagatgcagaaacaatctcagctttcaaatcttccactgtactaagggacttatgtgcttcattaagtttactttcttgttcagctattgtctgtctagctctctgaatctgttcccttgaaaagctcaattcttcaacaaggtcttcaagctgtctctgtagagcacacttttcttctaaaattagtcctagttcttccttgagtttttccttttgagagttagtatcttgcaattttatattcagttcatttattgccacattcattaactttatctgatcttcattaactgtaatatttgaatatgaccttaaagcattctccatttctcccttatgccgtgttttcatttcctccatctgtgccatgtgttgtcttattaattcttgtttcatttgcactatctgctgcccatacatctcatccagctctgcccggagttgttctaactttctttgtgtttcttgttccattcgttgtactatatcagtttcgaactggctgtctttatgatttctcttctgaagttcttcgactgtccccattaactgttttatttcttcagaagactgtctttctttttgcttagaattagtcagctctaatttcatgttttttatttcttggttcttttgcacaatctgttcttgtaattctcctagtaatttatcagcagttgttaatttatcctttagctcaagagttttcttttcttcttctattatttttgtgtttaattcttcaatgattgtctccttttcctgtatttcttctttatttgagttttctacttttttatcttgttccatttcatatactttaattttctcttgcaagaaactaatttgcattgtgaagtcttctttctttttctgataatcttctaataagtggtcttgttcttcaagctgctgttgatgagtgaggatctgttgtttggcttgtagtaagtctgcagctgtgctactatgagtgctgtttctcagagtttcactagcctgtaattgctgaaattgaatctgtaatttttgactctgttctgtcaactctaaaaattctctcattgtctcatccttttctcttcttgcttgttgtaaattagcagtgagctgggttataatgccatctctttgtttaatggcagcttcaaattcttgtaactgctgcagtccttcagtcccataggtaaccctcatttcttccagctctctgtttagctcttcaatctcatgctgcttcccagccaactcactttccatcatctctagatgagtcggactgtcttgtgctccttgttcagaataagaatcatcaacaccaaattcttcttcccttaataaatttgtaggctttcctgttctcatcacaaaactgcaaccatttactgaatacactgagttgctaaaccattcagagtacagaatagtttatagtctcctcaaattctggagtaaagaaatgacaatcacatctctgaactgcagtcatctgctgtggttgaaatttcactttccagttccacagagaagccctgctcatgactggttatttctccactatgtagagttctcattattgtagattcaggaatcacagttgattctactctctgagaactatttatgtac

SEQ ID NO: 14132 - RNA, 15949 nt, Homo sapiens
  source 1..15949: mol_type = other RNA
gctgggattacaggcatgagccaccgcacctggccttccctgcttcctctctagaatccaattagggatgtttgttactactcatattgattaaaacagttaacaaacttttttctttttaaaatgtgagatcagtgaactctggttttaagataatctgaaacaaggtccttgggagtaataaaattggtcacattctgtaaagcacattctgtttaggaatcaacttatctcaaattgtaactcggggcctaactatatgagatggctgaaaaaataccacatcgtctgttttcactaggtgatgccaaaatattttgctttatgtatattacagttctttttaaaacactggaagactcatgttaaactctaattgtgaaggcagaatctctgctaatttttcagattaaaattctctttgaaaaaatacagtctgtattcatgaattgtaaaatatgtgcttcagtgagcagagttagggaatccaggaacttgggtggggaaaaattacatctttatttgcactaataatttctaactgcaatttagtatttatttcaattatgaatttgggcagcattttattagcagtatccatgattttgtcaatagaaatctcagatattttcatattacagatgttacagatttcttgaagtatctagttacgaccccgagataaggctagtctaatgtttagtgaatagttttagacttcttaacagatttcatttttaatcacagactaattaattattgagatgcataaacaagtgtgattgcagaggcctactatcataaggaggcgtggtggtcaaacaatggcactgaactcagcttgatcagatcatttgtccatctgtttttttctccactgtctcttagagcagaatagccttgaatggcaagccatgctagctgaaaaaggtttttacccacaacctgccccttcaactaactgctttagagtacgtttgctatttttagaattcctcttattggaacccagcttctaatgtggaaaatttaagtatagttggctccttttatttgtgggttctgtatcctctgattcaaccaactgcaggttcaaaatactaaaaataaaaccccacaataaaaaaatacagtattagcaactatttacataatgttcacattgtattaggtatcaaataatctggagatgatttgaagtacacaggaggatgtatgtagactatctgcaaatagcacattgttttataagagacttaagcattcgcggactgtaatatccaagggggatcctggaactaatcccccacacatgccgagggatgactgaaattagaaatgttcaagcatgtacaactttctaccatgcctgtttgtgttggtataaatcatggaacatcaaataataagacaaaatcctccaggtgtaagcatcaaatactagtcctcttgctgttttagtgagttgccatgttattgaggaggactccagatgagaaataacattgcgatctgtattatctctgtgagagcctcccagtctgaatttggcttggacaacagggatactgtttaattcggctgcaatgtgattaagatcttttgagttaatgatttcttcatctttttagtgggccatggatttgtgagaacacatctttggaaacaagtaacactaactgtaatatagtaaatactgattaatcatgaaataccaatatagcttttaaaaaacactatgtagatgtaaagttgatacaaagacacatggaaaactttcaacagtattaactctaagattaggacaactttctctgaatctctcactcctacatatttgacataagtaatgagatgctatgtaccaagaactatggctcagttaaaaatgaagaaggttcaaatacagtgtggtgaaaatggtgaagtcatttttatttcagtacttgacaaaataccccataaaattcaaaacttctaccattatacaaaaataggtctctacaagtgatattatctgtcttcatcaccagtagaatatattaggcaaaacatgtaacttcagtagccttataagaaaagtgcaggacacctcgagctacacattcagcagtattgtaatgcgtaaaagtttaatcttttcacccatttgataaatacacaaggtttataatttaatgttttaaattagcattccacaaatatacaggtaattcaataattattgtgcatgaatacatacacaatgcttatatatacaaattccagtttgttttcatgtgctggcaagggatttgtatacaatcataagctgtgttcatattggtcccattgaatattcacaatacaaaagcacaaaagaaccattgatttacaaaaggaaatctatttaaaatcacttcaattaatgatgtttcaaaggattatcttctcatgccagcatgaaattgagtagttgaacctatgagagaaaaacaggaaattcaactgatttcaaattacattgctacctgtatcagacccaccagagttcacacaaaggaaattattattattctccatttttttaaagccctttttttccttaaaatgtcctcttcatacttaaactgagtctctccccactacccccaaggtggagtgttactctgttgcccaggctggaattcagtggtgtgatcttggctcactgcaacccccgcctcctgggttcaagtgattctcctgcctcagcctcctgagtagctgggactatccacacatgccaccatgtccagcaaatttttgtatttttagtggagacggggtttcaccatgttggccaggctagtctcgaactggttggtcttgaactcctgacctagtgatccgcctgcctcggccgcccaaagtgctgggattacaggcatgagccaccgcgcccagcccatatacttaagctgacttttaagagattttgaatatatatgtaaaaatcaccatgactggctctatggcaaggtaggtgagactaatatttagagtttttttaaagtgctctcaaagttggatgttctatacctcatacatttttgaaaaatcttttggtcttcaaaatctgggtcttgtgaaatttggatgctcaaaacaaaacaagcctaggcaaaccaacaaactcagctatgataataaaagtttcctattactacaagatgcttgggtgtaaacaaatgatttcttgaaggaagagataaactactcaatgattcaaagtctctgaatcaggagtgaactgaagtgagatagggaaaagaggttttccttccatgaacagggaatccacctttattttaaagtatgacttgttttttgtttttgaacaaagaaaaaataatccttacaaagtattttaaatgggatagtttttttcgatgatacataaaagcacaatatagtagcagggataatggttacattaagtgcttaaagtaagtgcttcctccttaactccacccgatttgcatgccttaccactttcttttttttttttttttctttgagacagggtctcgctctgctgcccaggctggagtgctgcggcacggccttaccactttctgccatgcgctacttaggaatacgttctccagttaggctctgtagactcagagtaccttgcacactggtgctcattgtgcattttgtgtcatcagtccgctgaatgaacatagtaggaaatcatttttgggaggagtgggatctggggtgataaatcatattttcacttaaattatttaaagtcagtttctctgctggttacaagagtttaagctttggctaacttaataattagctcatgcactaaactggaagctttgattatcctaatgagtgtgaaagaatttcaaagaaaggggagctgtgggtctcgcactgtggtgctgccaagatgtggttaaactcagagcacctgactgtatagttccaagtcgtctttgcagtgcctctagccgagtgatataatctgttagggctctgtcaggatcgtaattctgaagctgagaacatgctaaagaaccaggattgaaatcagctggagtgcctgggtacctattctgaaatggtaaaggggacctaatatagtccagatctgatcttgagcgatacgtagtatgtcttggttctccatataactccagcccaccagaagaatgataaaatgagtcagtcttttctgcaccttgattcagtccaaagccatctctgttaatattgatggaaacagaacctgtgactcgatgccaccgtcgaaccaaaaatttcattctggaaattgcaatggatactctgacggccgaccgaaacctggtgaagccctttgggcgattggtgatcacctctagatccgtgaaagctggctgcccccccatccgggcaagcagggccaaggtggcatcttcacattcctggaacccacccagtaacagcagcaggtatttcttctggtaaatgagagcctttcgaaaactttctgccctcaagtatttaccataaattctctttaaagtgacatgttcagaatcagggctcagagtttgaagtaaagagtcatttcttagttcagctttcagtttgtatacttcagcctctgcccttttcaaagatttctggagagtcaatttttctctgttccatacttctttttcagaggcaatgatggcttcaatgttggcaccaccattcaatgaaaacctggaagaattatctctaccagctcctgtctgtcgataccacctgatctgctcttccagcttcataaccatgttccttaagtcattcttctcttcagtcagttgactgatatgccctgtcagctcagcattttgtctcagtagtctttcagtcaatgagccacaagaagtacttggggacaccaagctgggctcttcaccttgctggccagttaatttctgtagttgtaaaataatttcatcaatattttcctgaacccaaatgaaatcttcatcatctgctgtttcaaactgtagtctctcagaggctttctggggtagaacctgtagttttgaagctacacattgaagcttttgtctgatcatttctaattcatgattacagccggttcctcctccattcatttcaatcaatttagcgtagtttgattcttttgtttctccttctattttctgttgaagaacccaatttctagttctatcactggttaagctccacgtggttggctcattaaggttctgatacagaattcttctactttctcgtttttcttctcgttctagttcttgcttctggaattcctgcatgattccttgtagtcgctgtccttcaaggtctaacttataaacttgttgtcttttctcttccagctggcgctgaagatcttccactttggactggagctcatgcatttttttctgtccctcagtgttggcctcctgttctgtctgcagtgttttcctgtgaacctgcctatctttttccatttgctgtcgtgtttgcaaagaatccagtttatatttttcagtctcatttaacaattctactatgcgactgtgtttttcctctagctgtttctgcagctctttcagtaggtcctctgagggcaagggtggccgagactgtccagtaccatcactgctctgcagctgtgcgtgcaattcccgctccctatctagggtactactcatttcccgaattcgaactttctcagattcaagaagtacctgaagctctaagtttcgaccttgttcttctgacaactgggcatcatatagcattctctgtgattctattttttgctgggattcgttcagtagttgtttctgttgttccaaaagtagatttagctgaagattcctttgtttctgactctcaagtgaaaacttcagatcctcaagttcttctttatcccgttcttcactgcgtcccaacttggctttctctttctccaaagcccactggagctctcttgattttttctgttcacttgctaatgtgtcattaagcaaatgtacttcatctgtcttatctttaacttccaacctgaaagcctccaattcttttaggtgtttatgctgtgccttgagtgttgtttctagttccaatttagtttgtgcaagctcactcttcagttcagcaaccaccattttctcagaactcagctgctcctgcagttccgttgctctgtctttcatactgctgagctccacttgcatctccagcatttgagactgcttctgctgtatattatattccaagagttcttggcttggtttctcactctcttgttctcttttcagagtaattttcctaccattcatttgtgcatgcagtgcctgaatttcagataacaaactccttctatctgctttctggaggcattccatagctgcttgatattcaacaccctgttcttgtattctctgttccaaacagtttagtaaaccaactgcatctgtagtacctagagctgtcagctccgtccgaaatgctgctagtaaaacactacgctcttctaagaaaacttgttgaagggcaagcagtagttcacctcgccagtctgagaagctctcatgagattgagaactatcataaacctcggcttctctttgcagttgcatctttgtaattaaatcctttagagatgagattgtattgatgtaagcttttctctcttctagccaaggttctgaaacctgctgaatagaatggtcctctccatcactatagggagactcagtgagagaaagcacctgcatgccttcattatggacagctctcagtaatccctttattttctttggaaaggaatctgttgcactttcactttcttctcctcggccttctgatgctatgtcaaatccctgactgtgtgtaagataaattccctgaccccagtctgatccagaatcactggagcatatttctctagtctggtaagcatcagaatgtgctagctcaggaattgaggatccctctttacttctcagacactgtatcactgccttcaaggtaccacattcctctttcagtaactgaacggcaacatagtgttccctctttaaggtttcagtttctgaaatatgtctggattccatgtccaaaatttcagcagcatgtagttcttgcatcttctcaattttttcagtaaactgactgattatttcagtaacttcttctgaggaacattcactctgtaaattaatttgtattcctgcatttttaacaagaatttgtggagtctgattgctgctactgatcttcagagtcccatctgtctgggatgcaatgctcttactcagttttataggaagtggctcaaacatgcaggcctttttgctttcttgtacctcagtctcatcttctttttctaaaatggacaatttctcttttgcctctgcgaggtgatccctaacttggcttaagtctttctgaagagatgtcatatttgtttcttttaccaaaagctcttcttgaagtttttcagccttttctttataactggcaagttctgctttggtagccactgattcagctctaagagcctcgagttcattaaaaaatccactttcttcattgctatgaaatagctcagtagttgtcttgagaacttcaacatcttgagggcttcttttcttttctttctctctctgttttttctcattgccctccaatagcttctgtagttctagcagcttcttttctttttctaaaacatttttttctgcaatttctacttgttctttttctaaaatcaaactagtatgcatttcaacaacctggctttctaattctgatattctcaaggttaatgctgatatatctgaccccaactcatcttctcttagttgatttaaattctgaatatttgttctttcaggttctgatgaaattgtttgattatcttgacagaattttgcatattcctgaactgcctcaagttggatttgactgacaagagcagcagccactttttcttcaactattttctgtaggtttacaatcttcttttgaagcatttctgtttcaaactggccttgttcttgcatgtcttttatttgtttataacactgggtaagttctaagtcctttgcactaacagtgctctcaagttgtagcaaccttgtttccaaattaattatggaacctttgccattttcttcaaaagatttgaagtatgtctgattttctagggatttaagagcatcctctgtaaggactacttctagttcaggtttgtctttgctcagatgatctatagccacgttaacactattctctggtatgctttgaatcttttccacactttcacgttctctctttaagctgaataattcctgtgttagctgattcattttaaaattggtttctttaagtacatttttcatgaaggtcatttcttcattagcggtttctacttgctgttccaaggccagcttttcagctataaccacatccaattgatgttttaaactgtctgcttcttctgagagggaatgagcattcattgatgtcttctgtccaatatttgccaattcctgttgaagtttttcaatcacttcattgagctgctctatttcttcttctctatttctcttcacacattcttgatcactcatcaaacattctatttgggtttcaagatcccttatcagttcatttttttcttcaataaccttgttatctgttgtaattttaagttgctgctggagtttcgtaacttgttcatttaattggtcaatttctacctctttttcctgtattatttgagcaaatttcccaaatagcacatgttggtcttgagtagacatggcatcagattcctttatggcaagtcccagtttctccatgtcatccttaaataatttgttttcctgttcaagttcttgtaggcgggtagtagattcctttttctgtatttctaattgcatatgtaattgttgaacttcttcattcttattttccagttcttctctaaactgttctaattgctcttctaagtttgtaatctctttttcctttctgtctatggcatctcgttcagcctgcaattgtacttctagggacaattctggtttagcttctacagctccaaagtgttttcggtcctctaccttttgaaaagtatctgcactcacaagaagcgcctgctccagttctcttactctgaactccagtttctctatttcttcattcctttcttgtatatccctttgaagctgctctttagagagcaaaagctcactgcatttgtctgttttttctttcagatgatttgctaactgttcaacctctctagtttgatgttcactgataggctggaatcgaggaacaaccttaagttgctgttctagtttctgtatttcctgttggaatacatctctctcatgttctctgtcaatggcttgctcatctaaaaattttctcattttttctaactgcttttccaatgcttggttttgctgtcttaaatccattagttcagtatttttttcttgttccagctctataaacctactgacttgttcttccacatctatttctagagctttcacttgtttttgaaggtcatcacgtactttttcagcttgacattgtacttctagtttttccttcattaatttttctgtctcctgtagtaattctgctcctggtgctgcatcgactgcagcatctactagtcgttgttcaactgggcctgcctctgctttcatagcttccttttgtctggacagtaattctctttcttcttggatctgctgttgctctgcctccaattcttgcaacctgttacttgcacataacaactcctgctcaagacgatctattatatcagttttttcctgaatttgcctttcaaaaagagttttttcatctgcatagccatcaatgacgccctcagccttactgagctccacagctagctgttctctggccctggactcctcatgaaggcgctctcgaagttcctcttggcacttaagggactctgttgcttcttgtttctgtctaaatgactcacgcatcaactctgtctgtgtcactttcgcatgttcaagctgactgctagtttcacttatggcttctaggagtttttcaactgctgcttgtagtcgagagctaatgttcagcataagttcttcattttcagggtctatttcagttccagcaaaaccactcctcacaagtcgttgtgacagctctgttccttcctcagttacttttgaccacatgttaatgtcatttcttggcatatcacttccagaataagagggaatggattcatctgtaactcttgtatgttcctcatggacacatgactttacagatgcctctgcttctgacctccaaattaggctggcagatgactggcttttactagatctatctagaatcccaaggacatggcgaccaattgtttcttcaacagctgctgttgtctttacaacttctaagaggatcttcaaaagtctattattagctttctggagtgcatacactgtctttcttgtttgagttccatactgactgcgttccatactgatgatccaatggggaagccaaaatcttaggggccaaattcctccatgcaagctttcattagacaaaatctcaggaggcacatcttcaggttttctgtctaattccttttctttaaatgtttgttcttcaacttctccttggttttcatttccattctgtgtttgcgtactgctgttgcgcagctcacaacacagcttctctcttccagctaaagacagctgctttagtgcttccagctcctctaaaagcaccctctctctctctgaaaccaggttttcattatctatggaggatctctgggctaattgtctattaagtctcttaatctcttcttgtagctgttcctggtcttctcgctgtctctccatttgccgcatatgtgcttgccttaacaattccgttgcctgttgatgttcttggtattgtcgtacaagttcctgtctcatatcttccaactgttcttcattcaacattagttgtctagaagcatccatgcttgacactgaaatctcatcatgaatagactgtctaactataaatgttttatctttggagaacatttcttctgaaatagtcagcacacagtcctttgattctggtatatcatggggatcactatttgataataaaatttcctttccatgttctcctaactctttactaagtggtttaaattcttctttaaatttcacatccactgtctcaaaagtctgaaaaccaatttgatcctgtgataatttcatttcattaaaataatgttgttcttgctgacacacagcatgtgcttgctttgatgatgcagtattttcttttcccccagatattctagacagttcagtttgttgagcaaatgctatactcattgacacaataaccttagctacttcttcttctaattgttcttggtattgtttttcaagcaacttaacgatatttgtttcctctttcactccaaattcaccagaaaactctattgtaccatcaatattctttttcacacaacttccagggtacattgttctctgtgcatcagattctgtaattaccaccgaatcaacaggtaagcttggcggaaccgtggactcactaacagcttgaagcctcttctgtaaacagtggatctctgcctcatagttttgttcagtttctttcaactgttgctgcaaagaggatatgaggctttctaattcttgaacttgttcttcaagtttagttttttcaagatcttgcagagaagataacttgcttttatgattgacatcaatgtcttccaaattggtcatctgagaatggattgataaaaactctgtttcctcttttggaaggttttcttctccaaattcaagtttcataccatctgtctgctgtccccagatcttgcttagtcgtgtttgaagtaccaagagtttgttgtattcttctgttactttgttgagaagagtgtgcatattttcttgaaagtcttgaacttcatatctataatcttgtaattctggatcttcattttcagaaatgtaatcaccagaattctctttgtcttctgcatttacttcacattttaaagcaggagtataatattcaccaaggacactgcataaagtctgtaaaaaataagaacattcttcagacactgccttttgaagttttccaatgagcagatgtaaaggctttccttcatcacctgtttcttgtgttttcatagtctgtagttctaactggtgtattttctgaagttccttgatcttttcctcttgagcaaaaataagctcttctttaagactgcaaagagctttatctttttcattttccatatattcacgaacctgatccacatgagttgaataaaccagagagaggcaaatgcgttgggcttccatctgtagccttaaatcattctgttctgatttaagtacattgagttctttctgaagtttatcattttcacttggttgagttgctctaagtgatgattcctttgttacagatggtaagtgatccaaaatcaactgttcttgcttactttcttctccaacagtcatattttcaaaagaaactttatcttccaccattatttttgattcttcaccaaaacttttatttactttagaaactgatccttcagcacccctgcttgtcatggtcacaactccatctaataaagagcttacttgagtatcacatgactgtacattttctgccctgttgtggttaataatgatttctagctctctacatctcaatgaaacttgttctttctcttgctttaaagatttaacttcttcatttagaaaactaatctcaccatgtttctgtttcaattgttcagaaagatcagacagtctctgtgacagctctaatttctctcgcttggttacctcaagtttttccatgagttctgttgtatccttttcaacaacctcacccatttccaatgtttctgctacaaaagttttgtcttcatcaaagacagaacttttcattttcactgtagttggatttattctttgcaaatgaagctcttcattaagtgctttaagtttacttttatactctaattcctgtttatttttactgtcttctaaatcatcttttactttgagaaggcaagcatactcctcttgtaactcttgatagttaacttcaaagtttttttcagcaaatgaaaaagtgttcctttgcttttcaatctcttcatttagctgaatacattgttgtttgaggtcctcattttcctctataagtatttctatttctttttcccacacagagtctttggatttggacttaatggagtctaagaaaatcaatctttcttcttggctaacaggagtatgtattttcaacatgtcttcaagggttttcttttcatctttaagaatgctattctctgcttcaagttgtgcaaatttttcttgaagatcattctctttttccttcatctgtttttctaacaattctgttttaagttgtaattcttgaacttcttgttcaagtgtacccttttctttttcttcttgtctgagtatttcaatttctttttgaagttcattgatttgaagagtcatttcttctgactttgaatttacaagagactgctgtaaatcttttagctttgaaatttccaaaattaattgattctgcttagttatcaaattgtccttttcaaactgcatggtttctatcttttgactcatttcattctgtaaaccatctatctgctgtttatagtgaatgcctaaattatctttaagtttttcaatatttattcgatgttcaatttctaaatcttccttcagtttggaaagctcttcttcgtgactaaatagaagctgtgttctcagcctctctaattcagcttcttgtgattcagccattctgtctaacacagcattcttttctttttctaacatttcaagttttatcttgtaatttgtaacttctgcttcatgttttaattctagttcctttctggattcagatgcagaaacaatctcagctttcaaatcttccactgtactaagggacttatgtgcttcattaagtttactttcttgttcagctattgtctgtctagctctctgaatctgttcccttgaaaagctcaattcttcaacaaggtcttcaagctgtctctgtagagcacacttttcttctaaaattagtcctagttcttccttgagtttttccttttgagagttagtatcttgcaattttatattcagttcatttattgccacattcattaactttatctgatcttcattaactgtaatatttgaatatgaccttaaagcattctccatttctcccttatgccgtgttttcatttcctccatctgtgccatgtgttgtcttattaattcttgtttcatttgcactatctgctgcccatacatctcatccagctctgcccggagttgttctaactttctttgtgtttcttgttccattcgttgtactatatcagtttcgaactggctgtctttatgatttctcttctgaagttcttcgactgtccccattaactgttttatttcttcagaagactgtctttctttttgcttagaattagtcagctctaatttcatgttttttatttcttggttcttttgcacaatctgttcttgtaattctcctagtaatttatcagcagttgttaatttatcctttagctcaagagttttcttttcttcttctattatttttgtgtttaattcttcaatgattgtctccttttcctgtatttcttctttatttgagttttctacttttttatcttgttccatttcatatactttaattttctcttgcaagaaactaatttgcattgtgaagtcttctttctttttctgataatcttctaataagtggtcttgttcttcaagctgctgttgatgagtgaggatctgttgtttggcttgtagtaagtctgcagctgtgctactatgagtgctgtttctcagagtttcactagcctgtaattgctgaaattgaatctgtaatttttgactctgttctgtcaactctaaaaattctctcattgtctcatccttttctcttcttgcttgttgtaaattagcagtgagctgggttataatgccatctctttgtttaatggcagcttcaaattcttgtaactgctgcagtccttcagtcccataggtaaccctcatttcttccagctctctgtttagctcttcaatctcatgctgcttcccagccaactcactttccatcatctctagatgagtcggactgtcttgtgctccttgttcagaataagaatcatcaacaccaaattcttcttcctctgaactgcagtcatctgctgtggttgaaatttcactttccagttccacagagaagccctgctcatgactggttatttctccactatgtagagttctcattattgtagattcaggaatcacagttgattctactctctgagaactatttatgtacatttcattacactgtgattgatcaatattcaaatcatggtgtgctgacacatcatgtttactgcttgacgtttttctcttttttttctgcttcttggaaggactctgcccatccgactgagcttttctttgtcgaaactgggcaagcttggctttgccggcctccagcttcttctgtctctcctcgtcctccatggcctctgcaaggaaggcaggggaaaacaggggttgaggggtggttggggatagaaaggaaaggtcgatttggacggaggtgggacggcaagctccacggcctagagagccgattcggtccggcgctcccccgcccgaagtggaagcagtctccgcgctcactggcggatcgtcctcagccgcacgggaagcgccgtcaccgccgccgccgccgccatcttcgtctccacgta

SEQ ID NO: 14133 - RNA, 15766 nt, Homo sapiens
  source 1..15766: mol_type = other RNA
gctgggattacaggcatgagccaccgcacctggccttccctgcttcctctctagaatccaattagggatgtttgttactactcatattgattaaaacagttaacaaacttttttctttttaaaatgtgagatcagtgaactctggttttaagataatctgaaacaaggtccttgggagtaataaaattggtcacattctgtaaagcacattctgtttaggaatcaacttatctcaaattgtaactcggggcctaactatatgagatggctgaaaaaataccacatcgtctgttttcactaggtgatgccaaaatattttgctttatgtatattacagttctttttaaaacactggaagactcatgttaaactctaattgtgaaggcagaatctctgctaatttttcagattaaaattctctttgaaaaaatacagtctgtattcatgaattgtaaaatatgtgcttcagtgagcagagttagggaatccaggaacttgggtggggaaaaattacatctttatttgcactaataatttctaactgcaatttagtatttatttcaattatgaatttgggcagcattttattagcagtatccatgattttgtcaatagaaatctcagatattttcatattacagatgttacagatttcttgaagtatctagttacgaccccgagataaggctagtctaatgtttagtgaatagttttagacttcttaacagatttcatttttaatcacagactaattaattattgagatgcataaacaagtgtgattgcagaggcctactatcataaggaggcgtggtggtcaaacaatggcactgaactcagcttgatcagatcatttgtccatctgtttttttctccactgtctcttagagcagaatagccttgaatggcaagccatgctagctgaaaaaggtttttacccacaacctgccccttcaactaactgctttagagtacgtttgctatttttagaattcctcttattggaacccagcttctaatgtggaaaatttaagtatagttggctccttttatttgtgggttctgtatcctctgattcaaccaactgcaggttcaaaatactaaaaataaaaccccacaataaaaaaatacagtattagcaactatttacataatgttcacattgtattaggtatcaaataatctggagatgatttgaagtacacaggaggatgtatgtagactatctgcaaatagcacattgttttataagagacttaagcattcgcggactgtaatatccaagggggatcctggaactaatcccccacacatgccgagggatgactgaaattagaaatgttcaagcatgtacaactttctaccatgcctgtttgtgttggtataaatcatggaacatcaaataataagacaaaatcctccaggtgtaagcatcaaatactagtcctcttgctgttttagtgagttgccatgttattgaggaggactccagatgagaaataacattgcgatctgtattatctctgtgagagcctcccagtctgaatttggcttggacaacagggatactgtttaattcggctgcaatgtgattaagatcttttgagttaatgatttcttcatctttttagtgggccatggatttgtgagaacacatctttggaaacaagtaacactaactgtaatatagtaaatactgattaatcatgaaataccaatatagcttttaaaaaacactatgtagatgtaaagttgatacaaagacacatggaaaactttcaacagtattaactctaagattaggacaactttctctgaatctctcactcctacatatttgacataagtaatgagatgctatgtaccaagaactatggctcagttaaaaatgaagaaggttcaaatacagtgtggtgaaaatggtgaagtcatttttatttcagtacttgacaaaataccccataaaattcaaaacttctaccattatacaaaaataggtctctacaagtgatattatctgtcttcatcaccagtagaatatattaggcaaaacatgtaacttcagtagccttataagaaaagtgcaggacacctcgagctacacattcagcagtattgtaatgcgtaaaagtttaatcttttcacccatttgataaatacacaaggtttataatttaatgttttaaattagcattccacaaatatacaggtaattcaataattattgtgcatgaatacatacacaatgcttatatatacaaattccagtttgttttcatgtgctggcaagggatttgtatacaatcataagctgtgttcatattggtcccattgaatattcacaatacaaaagcacaaaagaaccattgatttacaaaaggaaatctatttaaaatcacttcaattaatgatgtttcaaaggattatcttctcatgccagcatgaaattgagtagttgaacctatgagagaaaaacaggaaattcaactgatttcaaattacattgctacctgtatcagacccaccagagttcacacaaaggaaattattattattctccatttttttaaagccctttttttccttaaaatgtcctcttcatacttaaactgagtctctccccactacccccaaggtggagtgttactctgttgcccaggctggaattcagtggtgtgatcttggctcactgcaacccccgcctcctgggttcaagtgattctcctgcctcagcctcctgagtagctgggactatccacacatgccaccatgtccagcaaatttttgtatttttagtggagacggggtttcaccatgttggccaggctagtctcgaactggttggtcttgaactcctgacctagtgatccgcctgcctcggccgcccaaagtgctgggattacaggcatgagccaccgcgcccagcccatatacttaagctgacttttaagagattttgaatatatatgtaaaaatcaccatgactggctctatggcaaggtaggtgagactaatatttagagtttttttaaagtgctctcaaagttggatgttctatacctcatacatttttgaaaaatcttttggtcttcaaaatctgggtcttgtgaaatttggatgctcaaaacaaaacaagcctaggcaaaccaacaaactcagctatgataataaaagtttcctattactacaagatgcttgggtgtaaacaaatgatttcttgaaggaagagataaactactcaatgattcaaagtctctgaatcaggagtgaactgaagtgagatagggaaaagaggttttccttccatgaacagggaatccacctttattttaaagtatgacttgttttttgtttttgaacaaagaaaaaataatccttacaaagtattttaaatgggatagtttttttcgatgatacataaaagcacaatatagtagcagggataatggttacattaagtgcttaaagtaagtgcttcctccttaactccacccgatttgcatgccttaccactttcttttttttttttttttctttgagacagggtctcgctctgctgcccaggctggagtgctgcggcacggccttaccactttctgccatgcgctacttaggaatacgttctccagttaggctctgtagactcagagtaccttgcacactggtgctcattgtgcattttgtgtcatcagtccgctgaatgaacatagtaggaaatcatttttgggaggagtgggatctggggtgataaatcatattttcacttaaattatttaaagtcagtttctctgctggttacaagagtttaagctttggctaacttaataattagctcatgcactaaactggaagctttgattatcctaatgagtgtgaaagaatttcaaagaaaggggagctgtgggtctcgcactgtggtgctgccaagatgtggttaaactcagagcacctgactgtatagttccaagtcgtctttgcagtgcctctagccgagtgatataatctgttagggctctgtcaggatcgtaattctgaagctgagaacatgctaaagaaccaggattgaaatcagctggagtgcctgggtacctattctgaaatggtaaaggggacctaatatagtccagatctgatcttgagcgatacgtagtatgtcttggttctccatataactccagcccaccagaagaatgataaaatgagtcagtcttttctgcaccttgattcagtccaaagccatctctgttaatattgatggaaacagaacctgtgactcgatgccaccgtcgaaccaaaaatttcattctggaaattgcaatggatactctgacggccgaccgaaacctggtgaagccctttgggcgattggtgatcacctctagatccgtgaaagctggctgcccccccatccgggcaagcagggccaaggtggcatcttcacattcctggaacccacccagtaacagcagcaggtatttcttctggtaaatgagagcctttcgaaaactttctgccctcaagtatttaccataaattctctttaaagtgacatgttcagaatcagggctcagagtttgaagtaaagagtcatttcttagttcagctttcagtttgtatacttcagcctctgcccttttcaaagatttctggagagtcaatttttctctgttccatacttctttttcagaggcaatgatggcttcaatgttggcaccaccattcaatgaaaacctggaagaattatctctaccagctcctgtctgtcgataccacctgatctgctcttccagcttcataaccatgttccttaagtcattcttctcttcagtcagttgactgatatgccctgtcagctcagcattttgtctcagtagtctttcagtcaatgagccacaagaagtacttggggacaccaagctgggctcttcaccttgctggccagttaatttctgtagttgtaaaataatttcatcaatattttcctgaacccaaatgaaatcttcatcatctgctgtttcaaactgtagtctctcagaggctttctggggtagaacctgtagttttgaagctacacattgaagcttttgtctgatcatttctaattcatgattacagccggttcctcctccattcatttcaatcaatttagcgtagtttgattcttttgtttctccttctattttctgttgaagaacccaatttctagttctatcactggttaagctccacgtggttggctcattaaggttctgatacagaattcttctactttctcgtttttcttctcgttctagttcttgcttctggaattcctgcatgattccttgtagtcgctgtccttcaaggtctaacttataaacttgttgtcttttctcttccagctggcgctgaagatcttccactttggactggagctcatgcatttttttctgtccctcagtgttggcctcctgttctgtctgcagtgttttcctgtgaacctgcctatctttttccatttgctgtcgtgtttgcaaagaatccagtttatatttttcagtctcatttaacaattctactatgcgactgtgtttttcctctagctgtttctgcagctctttcagtaggtcctctgagggcaagggtggccgagactgtccagtaccatcactgctctgcagctgtgcgtgcaattcccgctccctatctagggtactactcatttcccgaattcgaactttctcagattcaagaagtacctgaagctctaagtttcgaccttgttcttctgacaactgggcatcatatagcattctctgtgattctattttttgctgggattcgttcagtagttgtttctgttgttccaaaagtagatttagctgaagattcctttgtttctgactctcaagtgaaaacttcagatcctcaagttcttctttatcccgttcttcactgcgtcccaacttggctttctctttctccaaagcccactggagctctcttgattttttctgttcacttgctaatgtgtcattaagcaaatgtacttcatctgtcttatctttaacttccaacctgaaagcctccaattcttttaggtgtttatgctgtgccttgagtgttgtttctagttccaatttagtttgtgcaagctcactcttcagttcagcaaccaccattttctcagaactcagctgctcctgcagttccgttgctctgtctttcatactgctgagctccacttgcatctccagcatttgagactgcttctgctgtatattatattccaagagttcttggcttggtttctcactctcttgttctcttttcagagtaattttcctaccattcatttgtgcatgcagtgcctgaatttcagataacaaactccttctatctgctttctggaggcattccatagctgcttgatattcaacaccctgttcttgtattctctgttccaaacagtttagtaaaccaactgcatctgtagtacctagagctgtcagctccgtccgaaatgctgctagtaaaacactacgctcttctaagaaaacttgttgaagggcaagcagtagttcacctcgccagtctgagaagctctcatgagattgagaactatcataaacctcggcttctctttgcagttgcatctttgtaattaaatcctttagagatgagattgtattgatgtaagcttttctctcttctagccaaggttctgaaacctgctgaatagaatggtcctctccatcactatagggagactcagtgagagaaagcacctgcatgccttcattatggacagctctcagtaatccctttattttctttggaaaggaatctgttgcactttcactttcttctcctcggccttctgatgctatgtcaaatccctgactgtgtgtaagataaattccctgaccccagtctgatccagaatcactggagcatatttctctagtctggtaagcatcagaatgtgctagctcaggaattgaggatccctctttacttctcagacactgtatcactgccttcaaggtaccacattcctctttcagtaactgaacggcaacatagtgttccctctttaaggtttcagtttctgaaatatgtctggattccatgtccaaaatttcagcagcatgtagttcttgcatcttctcaattttttcagtaaactgactgattatttcagtaacttcttctgaggaacattcactctgtaaattaatttgtattcctgcatttttaacaagaatttgtggagtctgattgctgctactgatcttcagagtcccatctgtctgggatgcaatgctcttactcagttttataggaagtggctcaaacatgcaggcctttttgctttcttgtacctcagtctcatcttctttttctaaaatggacaatttctcttttgcctctgcgaggtgatccctaacttggcttaagtctttctgaagagatgtcatatttgtttcttttaccaaaagctcttcttgaagtttttcagccttttctttataactggcaagttctgctttggtagccactgattcagctctaagagcctcgagttcattaaaaaatccactttcttcattgctatgaaatagctcagtagttgtcttgagaacttcaacatcttgagggcttcttttcttttctttctctctctgttttttctcattgccctccaatagcttctgtagttctagcagcttcttttctttttctaaaacatttttttctgcaatttctacttgttctttttctaaaatcaaactagtatgcatttcaacaacctggctttctaattctgatattctcaaggttaatgctgatatatctgaccccaactcatcttctcttagttgatttaaattctgaatatttgttctttcaggttctgatgaaattgtttgattatcttgacagaattttgcatattcctgaactgcctcaagttggatttgactgacaagagcagcagccactttttcttcaactattttctgtaggtttacaatcttcttttgaagcatttctgtttcaaactggccttgttcttgcatgtcttttatttgtttataacactgggtaagttctaagtcctttgcactaacagtgctctcaagttgtagcaaccttgtttccaaattaattatggaacctttgccattttcttcaaaagatttgaagtatgtctgattttctagggatttaagagcatcctctgtaaggactacttctagttcaggtttgtctttgctcagatgatctatagccacgttaacactattctctggtatgctttgaatcttttccacactttcacgttctctctttaagctgaataattcctgtgttagctgattcattttaaaattggtttctttaagtacatttttcatgaaggtcatttcttcattagcggtttctacttgctgttccaaggccagcttttcagctataaccacatccaattgatgttttaaactgtctgcttcttctgagagggaatgagcattcattgatgtcttctgtccaatatttgccaattcctgttgaagtttttcaatcacttcattgagctgctctatttcttcttctctatttctcttcacacattcttgatcactcatcaaacattctatttgggtttcaagatcccttatcagttcatttttttcttcaataaccttgttatctgttgtaattttaagttgctgctggagtttcgtaacttgttcatttaattggtcaatttctacctctttttcctgtattatttgagcaaatttcccaaatagcacatgttggtcttgagtagacatggcatcagattcctttatggcaagtcccagtttctccatgtcatccttaaataatttgttttcctgttcaagttcttgtaggcgggtagtagattcctttttctgtatttctaattgcatatgtaattgttgaacttcttcattcttattttccagttcttctctaaactgttctaattgctcttctaagtttgtaatctctttttcctttctgtctatggcatctcgttcagcctgcaattgtacttctagggacaattctggtttagcttctacagctccaaagtgttttcggtcctctaccttttgaaaagtatctgcactcacaagaagcgcctgctccagttctcttactctgaactccagtttctctatttcttcattcctttcttgtatatccctttgaagctgctctttagagagcaaaagctcactgcatttgtctgttttttctttcagatgatttgctaactgttcaacctctctagtttgatgttcactgataggctggaatcgaggaacaaccttaagttgctgttctagtttctgtatttcctgttggaatacatctctctcatgttctctgtcaatggcttgctcatctaaaaattttctcattttttctaactgcttttccaatgcttggttttgctgtcttaaatccattagttcagtatttttttcttgttccagctctataaacctactgacttgttcttccacatctatttctagagctttcacttgtttttgaaggtcatcacgtactttttcagcttgacattgtacttctagtttttccttcattaatttttctgtctcctgtagtaattctgctcctggtgctgcatcgactgcagcatctactagtcgttgttcaactgggcctgcctctgctttcatagcttccttttgtctggacagtaattctctttcttcttggatctgctgttgctctgcctccaattcttgcaacctgttacttgcacataacaactcctgctcaagacgatctattatatcagttttttcctgaatttgcctttcaaaaagagttttttcatctgcatagccatcaatgacgccctcagccttactgagctccacagctagctgttctctggccctggactcctcatgaaggcgctctcgaagttcctcttggcacttaagggactctgttgcttcttgtttctgtctaaatgactcacgcatcaactctgtctgtgtcactttcgcatgttcaagctgactgctagtttcacttatggcttctaggagtttttcaactgctgcttgtagtcgagagctaatgttcagcataagttcttcattttcagggtctatttcagttccagcaaaaccactcctcacaagtcgttgtgacagctctgttccttcctcagttacttttgaccacatgttaatgtcatttcttggcatatcacttccagaataagagggaatggattcatctgtaactcttgtatgttcctcatggacacatgactttacagatgcctctgcttctgacctccaaattaggctggcagatgactggcttttactagatctatctagaatcccaaggacatggcgaccaattgtttcttcaacagctgctgttgtctttacaacttctaagaggatcttcaaaagtctattattagctttctggagtgcatacctttcattagacaaaatctcaggaggcacatcttcaggttttctgtctaattccttttctttaaatgtttgttcttcaacttctccttggttttcatttccattctgggctaattgtctattaagtctcttaatctcttcttgtagctgttcctggtcttctcgctgtctctccatttgccgcatatgtgcttgccttaacaattccgttgcctgttgatgttcttggtattgtcgtacaagttcctgtctcatatcttccaactgttcttcattcaacattagttgtctagaagcatccatgcttgacactgaaatctcatcatgaatagactgtctaactataaatgttttatctttggagaacatttcttctgaaatagtcagcacacagtcctttgattctggtatatcatggggatcactatttgataataaaatttcctttccatgttctcctaactctttactaagtggtttaaattcttctttaaatttcacatccactgtctcaaaagtctgaaaaccaatttgatcctgtgataatttcatttcattaaaataatgttgttcttgctgacacacagcatgtgcttgctttgatgatgcagtattttcttttcccccagatattctagacagttcagtttgttgagcaaatgctatactcattgacacaataaccttagctacttcttcttctaattgttcttggtattgtttttcaagcaacttaacgatatttgtttcctctttcactccaaattcaccagaaaactctattgtaccatcaatattctttttcacacaacttccagggtacattgttctctgtgcatcagattctgtaattaccaccgaatcaacaggtaagcttggcggaaccgtggactcactaacagcttgaagcctcttctgtaaacagtggatctctgcctcatagttttgttcagtttctttcaactgttgctgcaaagaggatatgaggctttctaattcttgaacttgttcttcaagtttagttttttcaagatcttgcagagaagataacttgcttttatgattgacatcaatgtcttccaaattggtcatctgagaatggattgataaaaactctgtttcctcttttggaaggttttcttctccaaattcaagtttcataccatctgtctgctgtccccagatcttgcttagtcgtgtttgaagtaccaagagtttgttgtattcttctgttactttgttgagaagagtgtgcatattttcttgaaagtcttgaacttcatatctataatcttgtaattctggatcttcattttcagaaatgtaatcaccagaattctctttgtcttctgcatttacttcacattttaaagcaggagtataatattcaccaaggacactgcataaagtctgtaaaaaataagaacattcttcagacactgccttttgaagttttccaatgagcagatgtaaaggctttccttcatcacctgtttcttgtgttttcatagtctgtagttctaactggtgtattttctgaagttccttgatcttttcctcttgagcaaaaataagctcttctttaagactgcaaagagctttatctttttcattttccatatattcacgaacctgatccacatgagttgaataaaccagagagaggcaaatgcgttgggcttccatctgtagccttaaatcattctgttctgatttaagtacattgagttctttctgaagtttatcattttcacttggttgagttgctctaagtgatgattcctttgttacagatggtaagtgatccaaaatcaactgttcttgcttactttcttctccaacagtcatattttcaaaagaaactttatcttccaccattatttttgattcttcaccaaaacttttatttactttagaaactgatccttcagcacccctgcttgtcatggtcacaactccatctaataaagagcttacttgagtatcacatgactgtacattttctgccctgttgtggttaataatgatttctagctctctacatctcaatgaaacttgttctttctcttgctttaaagatttaacttcttcatttagaaaactaatctcaccatgtttctgtttcaattgttcagaaagatcagacagtctctgtgacagctctaatttctctcgcttggttacctcaagtttttccatgagttctgttgtatccttttcaacaacctcacccatttccaatgtttctgctacaaaagttttgtcttcatcaaagacagaacttttcattttcactgtagttggatttattctttgcaaatgaagctcttcattaagtgctttaagtttacttttatactctaattcctgtttatttttactgtcttctaaatcatcttttactttgagaaggcaagcatactcctcttgtaactcttgatagttaacttcaaagtttttttcagcaaatgaaaaagtgttcctttgcttttcaatctcttcatttagctgaatacattgttgtttgaggtcctcattttcctctataagtatttctatttctttttcccacacagagtctttggatttggacttaatggagtctaagaaaatcaatctttcttcttggctaacaggagtatgtattttcaacatgtcttcaagggttttcttttcatctttaagaatgctattctctgcttcaagttgtgcaaatttttcttgaagatcattctctttttccttcatctgtttttctaacaattctgttttaagttgtaattcttgaacttcttgttcaagtgtacccttttctttttcttcttgtctgagtatttcaatttctttttgaagttcattgatttgaagagtcatttcttctgactttgaatttacaagagactgctgtaaatcttttagctttgaaatttccaaaattaattgattctgcttagttatcaaattgtccttttcaaactgcatggtttctatcttttgactcatttcattctgtaaaccatctatctgctgtttatagtgaatgcctaaattatctttaagtttttcaatatttattcgatgttcaatttctaaatcttccttcagtttggaaagctcttcttcgtgactaaatagaagctgtgttctcagcctctctaattcagcttcttgtgattcagccattctgtctaacacagcattcttttctttttctaacatttcaagttttatcttgtaatttgtaacttctgcttcatgttttaattctagttcctttctggattcagatgcagaaacaatctcagctttcaaatcttccactgtactaagggacttatgtgcttcattaagtttactttcttgttcagctattgtctgtctagctctctgaatctgttcccttgaaaagctcaattcttcaacaaggtcttcaagctgtctctgtagagcacacttttcttctaaaattagtcctagttcttccttgagtttttccttttgagagttagtatcttgcaattttatattcagttcatttattgccacattcattaactttatctgatcttcattaactgtaatatttgaatatgaccttaaagcattctccatttctcccttatgccgtgttttcatttcctccatctgtgccatgtgttgtcttattaattcttgtttcatttgcactatctgctgcccatacatctcatccagctctgcccggagttgttctaactttctttgtgtttcttgttccattcgttgtactatatcagtttcgaactggctgtctttatgatttctcttctgaagttcttcgactgtccccattaactgttttatttcttcagaagactgtctttctttttgcttagaattagtcagctctaatttcatgttttttatttcttggttcttttgcacaatctgttcttgtaattctcctagtaatttatcagcagttgttaatttatcctttagctcaagagttttcttttcttcttctattatttttgtgtttaattcttcaatgattgtctccttttcctgtatttcttctttatttgagttttctacttttttatcttgttccatttcatatactttaattttctcttgcaagaaactaatttgcattgtgaagtcttctttctttttctgataatcttctaataagtggtcttgttcttcaagctgctgttgatgagtgaggatctgttgtttggcttgtagtaagtctgcagctgtgctactatgagtgctgtttctcagagtttcactagcctgtaattgctgaaattgaatctgtaatttttgactctgttctgtcaactctaaaaattctctcattgtctcatccttttctcttcttgcttgttgtaaattagcagtgagctgggttataatgccatctctttgtttaatggcagcttcaaattcttgtaactgctgcagtccttcagtcccataggtaaccctcatttcttccagctctctgtttagctcttcaatctcatgctgcttcccagccaactcactttccatcatctctagatgagtcggactgtcttgtgctccttgttcagaataagaatcatcaacaccaaattcttcttcccttaataaatttgtaggctttcctgttctcatcacaaaactgcaaccatttacctctgaactgcagtcatctgctgtggttgaaatttcactttccagttccacagagaagccctgctcatgactggttatttctccactatgtagagttctcattattgtagattcaggaatcacagttgattctactctctgagaactatttatgtacatttcattacactgtgattgatcaatattcaaatcatggtgtgctgacacatcatgtttactgcttgacgtttttctcttttttttctgcttcttggaaggactctgcccatccgactgagcttttctttgtcgaaactgggcaagcttggctttgccggcctccagcttcttctgtctctcctcgtcctccatggcctctgcaaggaaggcaggggaaaacaggggttgaggggtggttggggatagaaaggaaaggtcgatttggacggaggtgggacggcaagctccacggcctagagagccgattcggtccggcgctcccccgcccgaagtggaagcagtctccgcgctcactggcggatcgtcctcagccgcacgggaagcgccgtcaccgccgccgccgccgccatcttcgtctccacgta

SEQ ID NO: 14134 - RNA, 15907 nt, Homo sapiens
  source 1..15907: mol_type = other RNA
gctgggattacaggcatgagccaccgcacctggccttccctgcttcctctctagaatccaattagggatgtttgttactactcatattgattaaaacagttaacaaacttttttctttttaaaatgtgagatcagtgaactctggttttaagataatctgaaacaaggtccttgggagtaataaaattggtcacattctgtaaagcacattctgtttaggaatcaacttatctcaaattgtaactcggggcctaactatatgagatggctgaaaaaataccacatcgtctgttttcactaggtgatgccaaaatattttgctttatgtatattacagttctttttaaaacactggaagactcatgttaaactctaattgtgaaggcagaatctctgctaatttttcagattaaaattctctttgaaaaaatacagtctgtattcatgaattgtaaaatatgtgcttcagtgagcagagttagggaatccaggaacttgggtggggaaaaattacatctttatttgcactaataatttctaactgcaatttagtatttatttcaattatgaatttgggcagcattttattagcagtatccatgattttgtcaatagaaatctcagatattttcatattacagatgttacagatttcttgaagtatctagttacgaccccgagataaggctagtctaatgtttagtgaatagttttagacttcttaacagatttcatttttaatcacagactaattaattattgagatgcataaacaagtgtgattgcagaggcctactatcataaggaggcgtggtggtcaaacaatggcactgaactcagcttgatcagatcatttgtccatctgtttttttctccactgtctcttagagcagaatagccttgaatggcaagccatgctagctgaaaaaggtttttacccacaacctgccccttcaactaactgctttagagtacgtttgctatttttagaattcctcttattggaacccagcttctaatgtggaaaatttaagtatagttggctccttttatttgtgggttctgtatcctctgattcaaccaactgcaggttcaaaatactaaaaataaaaccccacaataaaaaaatacagtattagcaactatttacataatgttcacattgtattaggtatcaaataatctggagatgatttgaagtacacaggaggatgtatgtagactatctgcaaatagcacattgttttataagagacttaagcattcgcggactgtaatatccaagggggatcctggaactaatcccccacacatgccgagggatgactgaaattagaaatgttcaagcatgtacaactttctaccatgcctgtttgtgttggtataaatcatggaacatcaaataataagacaaaatcctccaggtgtaagcatcaaatactagtcctcttgctgttttagtgagttgccatgttattgaggaggactccagatgagaaataacattgcgatctgtattatctctgtgagagcctcccagtctgaatttggcttggacaacagggatactgtttaattcggctgcaatgtgattaagatcttttgagttaatgatttcttcatctttttagtgggccatggatttgtgagaacacatctttggaaacaagtaacactaactgtaatatagtaaatactgattaatcatgaaataccaatatagcttttaaaaaacactatgtagatgtaaagttgatacaaagacacatggaaaactttcaacagtattaactctaagattaggacaactttctctgaatctctcactcctacatatttgacataagtaatgagatgctatgtaccaagaactatggctcagttaaaaatgaagaaggttcaaatacagtgtggtgaaaatggtgaagtcatttttatttcagtacttgacaaaataccccataaaattcaaaacttctaccattatacaaaaataggtctctacaagtgatattatctgtcttcatcaccagtagaatatattaggcaaaacatgtaacttcagtagccttataagaaaagtgcaggacacctcgagctacacattcagcagtattgtaatgcgtaaaagtttaatcttttcacccatttgataaatacacaaggtttataatttaatgttttaaattagcattccacaaatatacaggtaattcaataattattgtgcatgaatacatacacaatgcttatatatacaaattccagtttgttttcatgtgctggcaagggatttgtatacaatcataagctgtgttcatattggtcccattgaatattcacaatacaaaagcacaaaagaaccattgatttacaaaaggaaatctatttaaaatcacttcaattaatgatgtttcaaaggattatcttctcatgccagcatgaaattgagtagttgaacctatgagagaaaaacaggaaattcaactgatttcaaattacattgctacctgtatcagacccaccagagttcacacaaaggaaattattattattctccatttttttaaagccctttttttccttaaaatgtcctcttcatacttaaactgagtctctccccactacccccaaggtggagtgttactctgttgcccaggctggaattcagtggtgtgatcttggctcactgcaacccccgcctcctgggttcaagtgattctcctgcctcagcctcctgagtagctgggactatccacacatgccaccatgtccagcaaatttttgtatttttagtggagacggggtttcaccatgttggccaggctagtctcgaactggttggtcttgaactcctgacctagtgatccgcctgcctcggccgcccaaagtgctgggattacaggcatgagccaccgcgcccagcccatatacttaagctgacttttaagagattttgaatatatatgtaaaaatcaccatgactggctctatggcaaggtaggtgagactaatatttagagtttttttaaagtgctctcaaagttggatgttctatacctcatacatttttgaaaaatcttttggtcttcaaaatctgggtcttgtgaaatttggatgctcaaaacaaaacaagcctaggcaaaccaacaaactcagctatgataataaaagtttcctattactacaagatgcttgggtgtaaacaaatgatttcttgaaggaagagataaactactcaatgattcaaagtctctgaatcaggagtgaactgaagtgagatagggaaaagaggttttccttccatgaacagggaatccacctttattttaaagtatgacttgttttttgtttttgaacaaagaaaaaataatccttacaaagtattttaaatgggatagtttttttcgatgatacataaaagcacaatatagtagcagggataatggttacattaagtgcttaaagtaagtgcttcctccttaactccacccgatttgcatgccttaccactttcttttttttttttttttctttgagacagggtctcgctctgctgcccaggctggagtgctgcggcacggccttaccactttctgccatgcgctacttaggaatacgttctccagttaggctctgtagactcagagtaccttgcacactggtgctcattgtgcattttgtgtcatcagtccgctgaatgaacatagtaggaaatcatttttgggaggagtgggatctggggtgataaatcatattttcacttaaattatttaaagtcagtttctctgctggttacaagagtttaagctttggctaacttaataattagctcatgcactaaactggaagctttgattatcctaatgagtgtgaaagaatttcaaagaaaggggagctgtgggtctcgcactgtggtgctgccaagatgtggttaaactcagagcacctgactgtatagttccaagtcgtctttgcagtgcctctagccgagtgatataatctgttagggctctgtcaggatcgtaattctgaagctgagaacatgctaaagaaccaggattgaaatcagctggagtgcctgggtacctattctgaaatggtaaaggggacctaatatagtccagatctgatcttgagcgatacgtagtatgtcttggttctccatataactccagcccaccagaagaatgataaaatgagtcagtcttttctgcaccttgattcagtccaaagccatctctgttaatattgatggaaacagaacctgtgactcgatgccaccgtcgaaccaaaaatttcattctggaaattgcaatggatactctgacggccgaccgaaacctggtgaagccctttgggcgattggtgatcacctctagatccgtgaaagctggctgcccccccatccgggcaagcagggccaaggtggcatcttcacattcctggaacccacccagtaacagcagcaggtatttcttctggtaaatgagagcctttcgaaaactttctgccctcaagtatttaccataaattctctttaaagtgacatgttcagaatcagggctcagagtttgaagtaaagagtcatttcttagttcagctttcagtttgtatacttcagcctctgcccttttcaaagatttctggagagtcaatttttctctgttccatacttctttttcagaggcaatgatggcttcaatgttggcaccaccattcaatgaaaacctggaagaattatctctaccagctcctgtctgtcgataccacctgatctgctcttccagcttcataaccatgttccttaagtcattcttctcttcagtcagttgactgatatgccctgtcagctcagcattttgtctcagtagtctttcagtcaatgagccacaagaagtacttggggacaccaagctgggctcttcaccttgctggccagttaatttctgtagttgtaaaataatttcatcaatattttcctgaacccaaatgaaatcttcatcatctgctgtttcaaactgtagtctctcagaggctttctggggtagaacctgtagttttgaagctacacattgaagcttttgtctgatcatttctaattcatgattacagccggttcctcctccattcatttcaatcaatttagcgtagtttgattcttttgtttctccttctattttctgttgaagaacccaatttctagttctatcactggttaagctccacgtggttggctcattaaggttctgatacagaattcttctactttctcgtttttcttctcgttctagttcttgcttctggaattcctgcatgattccttgtagtcgctgtccttcaaggtctaacttataaacttgttgtcttttctcttccagctggcgctgaagatcttccactttggactggagctcatgcatttttttctgtccctcagtgttggcctcctgttctgtctgcagtgttttcctgtgaacctgcctatctttttccatttgctgtcgtgtttgcaaagaatccagtttatatttttcagtctcatttaacaattctactatgcgactgtgtttttcctctagctgtttctgcagctctttcagtaggtcctctgagggcaagggtggccgagactgtccagtaccatcactgctctgcagctgtgcgtgcaattcccgctccctatctagggtactactcatttcccgaattcgaactttctcagattcaagaagtacctgaagctctaagtttcgaccttgttcttctgacaactgggcatcatatagcattctctgtgattctattttttgctgggattcgttcagtagttgtttctgttgttccaaaagtagatttagctgaagattcctttgtttctgactctcaagtgaaaacttcagatcctcaagttcttctttatcccgttcttcactgcgtcccaacttggctttctctttctccaaagcccactggagctctcttgattttttctgttcacttgctaatgtgtcattaagcaaatgtacttcatctgtcttatctttaacttccaacctgaaagcctccaattcttttaggtgtttatgctgtgccttgagtgttgtttctagttccaatttagtttgtgcaagctcactcttcagttcagcaaccaccattttctcagaactcagctgctcctgcagttccgttgctctgtctttcatactgctgagctccacttgcatctccagcatttgagactgcttctgctgtatattatattccaagagttcttggcttggtttctcactctcttgttctcttttcagagtaattttcctaccattcatttgtgcatgcagtgcctgaatttcagataacaaactccttctatctgctttctggaggcattccatagctgcttgatattcaacaccctgttcttgtattctctgttccaaacagtttagtaaaccaactgcatctgtagtacctagagctgtcagctccgtccgaaatgctgctagtaaaacactacgctcttctaagaaaacttgttgaagggcaagcagtagttcacctcgccagtctgagaagctctcatgagattgagaactatcataaacctcggcttctctttgcagttgcatctttgtaattaaatcctttagagatgagattgtattgatgtaagcttttctctcttctagccaaggttctgaaacctgctgaatagaatggtcctctccatcactatagggagactcagtgagagaaagcacctgcatgccttcattatggacagctctcagtaatccctttattttctttggaaaggaatctgttgcactttcactttcttctcctcggccttctgatgctatgtcaaatccctgactgtgtgtaagataaattccctgaccccagtctgatccagaatcactggagcatatttctctagtctggtaagcatcagaatgtgctagctcaggaattgaggatccctctttacttctcagacactgtatcactgccttcaaggtaccacattcctctttcagtaactgaacggcaacatagtgttccctctttaaggtttcagtttctgaaatatgtctggattccatgtccaaaatttcagcagcatgtagttcttgcatcttctcaattttttcagtaaactgactgattatttcagtaacttcttctgaggaacattcactctgtaaattaatttgtattcctgcatttttaacaagaatttgtggagtctgattgctgctactgatcttcagagtcccatctgtctgggatgcaatgctcttactcagttttataggaagtggctcaaacatgcaggcctttttgctttcttgtacctcagtctcatcttctttttctaaaatggacaatttctcttttgcctctgcgaggtgatccctaacttggcttaagtctttctgaagagatgtcatatttgtttcttttaccaaaagctcttcttgaagtttttcagccttttctttataactggcaagttctgctttggtagccactgattcagctctaagagcctcgagttcattaaaaaatccactttcttcattgctatgaaatagctcagtagttgtcttgagaacttcaacatcttgagggcttcttttcttttctttctctctctgttttttctcattgccctccaatagcttctgtagttctagcagcttcttttctttttctaaaacatttttttctgcaatttctacttgttctttttctaaaatcaaactagtatgcatttcaacaacctggctttctaattctgatattctcaaggttaatgctgatatatctgaccccaactcatcttctcttagttgatttaaattctgaatatttgttctttcaggttctgatgaaattgtttgattatcttgacagaattttgcatattcctgaactgcctcaagttggatttgactgacaagagcagcagccactttttcttcaactattttctgtaggtttacaatcttcttttgaagcatttctgtttcaaactggccttgttcttgcatgtcttttatttgtttataacactgggtaagttctaagtcctttgcactaacagtgctctcaagttgtagcaaccttgtttccaaattaattatggaacctttgccattttcttcaaaagatttgaagtatgtctgattttctagggatttaagagcatcctctgtaaggactacttctagttcaggtttgtctttgctcagatgatctatagccacgttaacactattctctggtatgctttgaatcttttccacactttcacgttctctctttaagctgaataattcctgtgttagctgattcattttaaaattggtttctttaagtacatttttcatgaaggtcatttcttcattagcggtttctacttgctgttccaaggccagcttttcagctataaccacatccaattgatgttttaaactgtctgcttcttctgagagggaatgagcattcattgatgtcttctgtccaatatttgccaattcctgttgaagtttttcaatcacttcattgagctgctctatttcttcttctctatttctcttcacacattcttgatcactcatcaaacattctatttgggtttcaagatcccttatcagttcatttttttcttcaataaccttgttatctgttgtaattttaagttgctgctggagtttcgtaacttgttcatttaattggtcaatttctacctctttttcctgtattatttgagcaaatttcccaaatagcacatgttggtcttgagtagacatggcatcagattcctttatggcaagtcccagtttctccatgtcatccttaaataatttgttttcctgttcaagttcttgtaggcgggtagtagattcctttttctgtatttctaattgcatatgtaattgttgaacttcttcattcttattttccagttcttctctaaactgttctaattgctcttctaagtttgtaatctctttttcctttctgtctatggcatctcgttcagcctgcaattgtacttctagggacaattctggtttagcttctacagctccaaagtgttttcggtcctctaccttttgaaaagtatctgcactcacaagaagcgcctgctccagttctcttactctgaactccagtttctctatttcttcattcctttcttgtatatccctttgaagctgctctttagagagcaaaagctcactgcatttgtctgttttttctttcagatgatttgctaactgttcaacctctctagtttgatgttcactgataggctggaatcgaggaacaaccttaagttgctgttctagtttctgtatttcctgttggaatacatctctctcatgttctctgtcaatggcttgctcatctaaaaattttctcattttttctaactgcttttccaatgcttggttttgctgtcttaaatccattagttcagtatttttttcttgttccagctctataaacctactgacttgttcttccacatctatttctagagctttcacttgtttttgaaggtcatcacgtactttttcagcttgacattgtacttctagtttttccttcattaatttttctgtctcctgtagtaattctgctcctggtgctgcatcgactgcagcatctactagtcgttgttcaactgggcctgcctctgctttcatagcttccttttgtctggacagtaattctctttcttcttggatctgctgttgctctgcctccaattcttgcaacctgttacttgcacataacaactcctgctcaagacgatctattatatcagttttttcctgaatttgcctttcaaaaagagttttttcatctgcatagccatcaatgacgccctcagccttactgagctccacagctagctgttctctggccctggactcctcatgaaggcgctctcgaagttcctcttggcacttaagggactctgttgcttcttgtttctgtctaaatgactcacgcatcaactctgtctgtgtcactttcgcatgttcaagctgactgctagtttcacttatggcttctaggagtttttcaactgctgcttgtagtcgagagctaatgttcagcataagttcttcattttcagggtctatttcagttccagcaaaaccactcctcacaagtcgttgtgacagctctgttccttcctcagttacttttgaccacatgttaatgtcatttcttggcatatcacttccagaataagagggaatggattcatctgtaactcttgtatgttcctcatggacacatgactttacagatgcctctgcttctgacctccaaattaggctggcagatgactggcttttactagatctatctagaatcccaaggacatggcgaccaattgtttcttcaacagctgctgttgtctttacaacttctaagaggatcttcaaaagtctattattagctttctggagtgcatacctttcattagacaaaatctcaggaggcacatcttcaggttttctgtctaattccttttctttaaatgtttgttcttcaacttctccttggttttcatttccattctgtgtttgcgtactgctgttgcgcagctcacaacacagcttctctcttccagctaaagacagctgctttagtgcttccagctcctctaaaagcaccctctctctctctgaaaccaggttttcattatctatggaggatctctgggctaattgtctattaagtctcttaatctcttcttgtagctgttcctggtcttctcgctgtctctccatttgccgcatatgtgcttgccttaacaattccgttgcctgttgatgttcttggtattgtcgtacaagttcctgtctcatatcttccaactgttcttcattcaacattagttgtctagaagcatccatgcttgacactgaaatctcatcatgaatagactgtctaactataaatgttttatctttggagaacatttcttctgaaatagtcagcacacagtcctttgattctggtatatcatggggatcactatttgataataaaatttcctttccatgttctcctaactctttactaagtggtttaaattcttctttaaatttcacatccactgtctcaaaagtctgaaaaccaatttgatcctgtgataatttcatttcattaaaataatgttgttcttgctgacacacagcatgtgcttgctttgatgatgcagtattttcttttcccccagatattctagacagttcagtttgttgagcaaatgctatactcattgacacaataaccttagctacttcttcttctaattgttcttggtattgtttttcaagcaacttaacgatatttgtttcctctttcactccaaattcaccagaaaactctattgtaccatcaatattctttttcacacaacttccagggtacattgttctctgtgcatcagattctgtaattaccaccgaatcaacaggtaagcttggcggaaccgtggactcactaacagcttgaagcctcttctgtaaacagtggatctctgcctcatagttttgttcagtttctttcaactgttgctgcaaagaggatatgaggctttctaattcttgaacttgttcttcaagtttagttttttcaagatcttgcagagaagataacttgcttttatgattgacatcaatgtcttccaaattggtcatctgagaatggattgataaaaactctgtttcctcttttggaaggttttcttctccaaattcaagtttcataccatctgtctgctgtccccagatcttgcttagtcgtgtttgaagtaccaagagtttgttgtattcttctgttactttgttgagaagagtgtgcatattttcttgaaagtcttgaacttcatatctataatcttgtaattctggatcttcattttcagaaatgtaatcaccagaattctctttgtcttctgcatttacttcacattttaaagcaggagtataatattcaccaaggacactgcataaagtctgtaaaaaataagaacattcttcagacactgccttttgaagttttccaatgagcagatgtaaaggctttccttcatcacctgtttcttgtgttttcatagtctgtagttctaactggtgtattttctgaagttccttgatcttttcctcttgagcaaaaataagctcttctttaagactgcaaagagctttatctttttcattttccatatattcacgaacctgatccacatgagttgaataaaccagagagaggcaaatgcgttgggcttccatctgtagccttaaatcattctgttctgatttaagtacattgagttctttctgaagtttatcattttcacttggttgagttgctctaagtgatgattcctttgttacagatggtaagtgatccaaaatcaactgttcttgcttactttcttctccaacagtcatattttcaaaagaaactttatcttccaccattatttttgattcttcaccaaaacttttatttactttagaaactgatccttcagcacccctgcttgtcatggtcacaactccatctaataaagagcttacttgagtatcacatgactgtacattttctgccctgttgtggttaataatgatttctagctctctacatctcaatgaaacttgttctttctcttgctttaaagatttaacttcttcatttagaaaactaatctcaccatgtttctgtttcaattgttcagaaagatcagacagtctctgtgacagctctaatttctctcgcttggttacctcaagtttttccatgagttctgttgtatccttttcaacaacctcacccatttccaatgtttctgctacaaaagttttgtcttcatcaaagacagaacttttcattttcactgtagttggatttattctttgcaaatgaagctcttcattaagtgctttaagtttacttttatactctaattcctgtttatttttactgtcttctaaatcatcttttactttgagaaggcaagcatactcctcttgtaactcttgatagttaacttcaaagtttttttcagcaaatgaaaaagtgttcctttgcttttcaatctcttcatttagctgaatacattgttgtttgaggtcctcattttcctctataagtatttctatttctttttcccacacagagtctttggatttggacttaatggagtctaagaaaatcaatctttcttcttggctaacaggagtatgtattttcaacatgtcttcaagggttttcttttcatctttaagaatgctattctctgcttcaagttgtgcaaatttttcttgaagatcattctctttttccttcatctgtttttctaacaattctgttttaagttgtaattcttgaacttcttgttcaagtgtacccttttctttttcttcttgtctgagtatttcaatttctttttgaagttcattgatttgaagagtcatttcttctgactttgaatttacaagagactgctgtaaatcttttagctttgaaatttccaaaattaattgattctgcttagttatcaaattgtccttttcaaactgcatggtttctatcttttgactcatttcattctgtaaaccatctatctgctgtttatagtgaatgcctaaattatctttaagtttttcaatatttattcgatgttcaatttctaaatcttccttcagtttggaaagctcttcttcgtgactaaatagaagctgtgttctcagcctctctaattcagcttcttgtgattcagccattctgtctaacacagcattcttttctttttctaacatttcaagttttatcttgtaatttgtaacttctgcttcatgttttaattctagttcctttctggattcagatgcagaaacaatctcagctttcaaatcttccactgtactaagggacttatgtgcttcattaagtttactttcttgttcagctattgtctgtctagctctctgaatctgttcccttgaaaagctcaattcttcaacaaggtcttcaagctgtctctgtagagcacacttttcttctaaaattagtcctagttcttccttgagtttttccttttgagagttagtatcttgcaattttatattcagttcatttattgccacattcattaactttatctgatcttcattaactgtaatatttgaatatgaccttaaagcattctccatttctcccttatgccgtgttttcatttcctccatctgtgccatgtgttgtcttattaattcttgtttcatttgcactatctgctgcccatacatctcatccagctctgcccggagttgttctaactttctttgtgtttcttgttccattcgttgtactatatcagtttcgaactggctgtctttatgatttctcttctgaagttcttcgactgtccccattaactgttttatttcttcagaagactgtctttctttttgcttagaattagtcagctctaatttcatgttttttatttcttggttcttttgcacaatctgttcttgtaattctcctagtaatttatcagcagttgttaatttatcctttagctcaagagttttcttttcttcttctattatttttgtgtttaattcttcaatgattgtctccttttcctgtatttcttctttatttgagttttctacttttttatcttgttccatttcatatactttaattttctcttgcaagaaactaatttgcattgtgaagtcttctttctttttctgataatcttctaataagtggtcttgttcttcaagctgctgttgatgagtgaggatctgttgtttggcttgtagtaagtctgcagctgtgctactatgagtgctgtttctcagagtttcactagcctgtaattgctgaaattgaatctgtaatttttgactctgttctgtcaactctaaaaattctctcattgtctcatccttttctcttcttgcttgttgtaaattagcagtgagctgggttataatgccatctctttgtttaatggcagcttcaaattcttgtaactgctgcagtccttcagtcccataggtaaccctcatttcttccagctctctgtttagctcttcaatctcatgctgcttcccagccaactcactttccatcatctctagatgagtcggactgtcttgtgctccttgttcagaataagaatcatcaacaccaaattcttcttcccttaataaatttgtaggctttcctgttctcatcacaaaactgcaaccatttacctctgaactgcagtcatctgctgtggttgaaatttcactttccagttccacagagaagccctgctcatgactggttatttctccactatgtagagttctcattattgtagattcaggaatcacagttgattctactctctgagaactatttatgtacatttcattacactgtgattgatcaatattcaaatcatggtgtgctgacacatcatgtttactgcttgacgtttttctcttttttttctgcttcttggaaggactctgcccatccgactgagcttttctttgtcgaaactgggcaagcttggctttgccggcctccagcttcttctgtctctcctcgtcctccatggcctctgcaaggaaggcaggggaaaacaggggttgaggggtggttggggatagaaaggaaaggtcgatttggacggaggtgggacggcaagctccacggcctagagagccgattcggtccggcgctcccccgcccgaagtggaagcagtctccgcgctcactggcggatcgtcctcagccgcacgggaagcgccgtcaccgccgccgccgccgccatcttcgtctccacgta

SEQ ID NO: 14135 - RNA, 10874 nt, Homo sapiens
  source 1..10874: mol_type = other RNA
gctgggattacaggcatgagccaccgcacctggccttccctgcttcctctctagaatccaattagggatgtttgttactactcatattgattaaaacagttaacaaacttttttctttttaaaatgtgagatcagtgaactctggttttaagataatctgaaacaaggtccttgggagtaataaaattggtcacattctgtaaagcacattctgtttaggaatcaacttatctcaaattgtaactcggggcctaactatatgagatggctgaaaaaataccacatcgtctgttttcactaggtgatgccaaaatattttgctttatgtatattacagttctttttaaaacactggaagactcatgttaaactctaattgtgaaggcagaatctctgctaatttttcagattaaaattctctttgaaaaaatacagtctgtattcatgaattgtaaaatatgtgcttcagtgagcagagttagggaatccaggaacttgggtggggaaaaattacatctttatttgcactaataatttctaactgcaatttagtatttatttcaattatgaatttgggcagcattttattagcagtatccatgattttgtcaatagaaatctcagatattttcatattacagatgttacagatttcttgaagtatctagttacgaccccgagataaggctagtctaatgtttagtgaatagttttagacttcttaacagatttcatttttaatcacagactaattaattattgagatgcataaacaagtgtgattgcagaggcctactatcataaggaggcgtggtggtcaaacaatggcactgaactcagcttgatcagatcatttgtccatctgtttttttctccactgtctcttagagcagaatagccttgaatggcaagccatgctagctgaaaaaggtttttacccacaacctgccccttcaactaactgctttagagtacgtttgctatttttagaattcctcttattggaacccagcttctaatgtggaaaatttaagtatagttggctccttttatttgtgggttctgtatcctctgattcaaccaactgcaggttcaaaatactaaaaataaaaccccacaataaaaaaatacagtattagcaactatttacataatgttcacattgtattaggtatcaaataatctggagatgatttgaagtacacaggaggatgtatgtagactatctgcaaatagcacattgttttataagagacttaagcattcgcggactgtaatatccaagggggatcctggaactaatcccccacacatgccgagggatgactgaaattagaaatgttcaagcatgtacaactttctaccatgcctgtttgtgttggtataaatcatggaacatcaaataataagacaaaatcctccaggtgtaagcatcaaatactagtcctcttgctgttttagtgagttgccatgttattgaggaggactccagatgagaaataacattgcgatctgtattatctctgtgagagcctcccagtctgaatttggcttggacaacagggatactgtttaattcggctgcaatgtgattaagatcttttgagttaatgatttcttcatctttttagtgggccatggatttgtgagaacacatctttggaaacaagtaacactaactgtaatatagtaaatactgattaatcatgaaataccaatatagcttttaaaaaacactatgtagatgtaaagttgatacaaagacacatggaaaactttcaacagtattaactctaagattaggacaactttctctgaatctctcactcctacatatttgacataagtaatgagatgctatgtaccaagaactatggctcagttaaaaatgaagaaggttcaaatacagtgtggtgaaaatggtgaagtcatttttatttcagtacttgacaaaataccccataaaattcaaaacttctaccattatacaaaaataggtctctacaagtgatattatctgtcttcatcaccagtagaatatattaggcaaaacatgtaacttcagtagccttataagaaaagtgcaggacacctcgagctacacattcagcagtattgtaatgcgtaaaagtttaatcttttcacccatttgataaatacacaaggtttataatttaatgttttaaattagcattccacaaatatacaggtaattcaataattattgtgcatgaatacatacacaatgcttatatatacaaattccagtttgttttcatgtgctggcaagggatttgtatacaatcataagctgtgttcatattggtcccattgaatattcacaatacaaaagcacaaaagaaccattgatttacaaaaggaaatctatttaaaatcacttcaattaatgatgtttcaaaggattatcttctcatgccagcatgaaattgagtagttgaacctatgagagaaaaacaggaaattcaactgatttcaaattacattgctacctgtatcagacccaccagagttcacacaaaggaaattattattattctccatttttttaaagccctttttttccttaaaatgtcctcttcatacttaaactgagtctctccccactacccccaaggtggagtgttactctgttgcccaggctggaattcagtggtgtgatcttggctcactgcaacccccgcctcctgggttcaagtgattctcctgcctcagcctcctgagtagctgggactatccacacatgccaccatgtccagcaaatttttgtatttttagtggagacggggtttcaccatgttggccaggctagtctcgaactggttggtcttgaactcctgacctagtgatccgcctgcctcggccgcccaaagtgctgggattacaggcatgagccaccgcgcccagcccatatacttaagctgacttttaagagattttgaatatatatgtaaaaatcaccatgactggctctatggcaaggtaggtgagactaatatttagagtttttttaaagtgctctcaaagttggatgttctatacctcatacatttttgaaaaatcttttggtcttcaaaatctgggtcttgtgaaatttggatgctcaaaacaaaacaagcctaggcaaaccaacaaactcagctatgataataaaagtttcctattactacaagatgcttgggtgtaaacaaatgatttcttgaaggaagagataaactactcaatgattcaaagtctctgaatcaggagtgaactgaagtgagatagggaaaagaggttttccttccatgaacagggaatccacctttattttaaagtatgacttgttttttgtttttgaacaaagaaaaaataatccttacaaagtattttaaatgggatagtttttttcgatgatacataaaagcacaatatagtagcagggataatggttacattaagtgcttaaagtaagtgcttcctccttaactccacccgatttgcatgccttaccactttcttttttttttttttttctttgagacagggtctcgctctgctgcccaggctggagtgctgcggcacggccttaccactttctgccatgcgctacttaggaatacgttctccagttaggctctgtagactcagagtaccttgcacactggtgctcattgtgcattttgtgtcatcagtccgctgaatgaacatagtaggaaatcatttttgggaggagtgggatctggggtgataaatcatattttcacttaaattatttaaagtcagtttctctgctggttacaagagtttaagctttggctaacttaataattagctcatgcactaaactggaagctttgattatcctaatgagtgtgaaagaatttcaaagaaaggggagctgtgggtctcgcactgtggtgctgccaagatgtggttaaactcagagcacctgactgtatagttccaagtcgtctttgcagtgcctctagccgagtgatataatctgttagggctctgtcaggatcgtaattctgaagctgagaacatgctaaagaaccaggattgaaatcagctggagtgcctgggtacctattctgaaatggtaaaggggacctaatatagtccagatctgatcttgagcgatacgtagtatgtcttggttctccatataactccagcccaccagaagaatgataaaatgagtcagtcttttctgcaccttgattcagtccaaagccatctctgttaatattgatggaaacagaacctgtgactcgatgccaccgtcgaaccaaaaatttcattctggaaattgcaatggatactctgacggccgaccgaaacctggtgaagccctttgggcgattggtgatcacctctagatccgtgaaagctggctgcccccccatccgggcaagcagggccaaggtggcatcttcacattcctggaacccacccagtaacagcagcaggtatttcttctggtaaatgagagcctttcgaaaactttctgccctcaagtatttaccataaattctctttaaagtgacatgttcagaatcagggctcagagtttgaagtaaagagtcatttcttagttcagctttcagtttgtatacttcagcctctgcccttttcaaagatttctggagagtcaatttttctctgttccatacttctttttcagaggcaatgatggcttcaatgttggcaccaccattcaatgaaaacctggaagaattatctctaccagctcctgtctgtcgataccacctgatctgctcttccagcttcataaccatgttccttaagtcattcttctcttcagtcagttgactgatatgccctgtcagctcagcattttgtctcagtagtctttcagtcaatgagccacaagaagtacttggggacaccaagctgggctcttcaccttgctggccagttaatttctgtagttgtaaaataatttcatcaatattttcctgaacccaaatgaaatcttcatcatctgctgtttcaaactgtagtctctcagaggctttctggggtagaacctgtagttttgaagctacacattgaagcttttgtctgatcatttctaattcatgattacagccggttcctcctccattcatttcaatcaatttagcgtagtttgattcttttgtttctccttctattttctgttgaagaacccaatttctagttctatcactggttaagctccacgtggttggctcattaaggttctgatacagaattcttctactttctcgtttttcttctcgttctagttcttgcttctggaattcctgcatgattccttgtagtcgctgtccttcaaggtctaacttataaacttgttgtcttttctcttccagctggcgctgaagatcttccactttggactggagctcatgcatttttttctgtccctcagtgttggcctcctgttctgtctgcagtgttttcctgtgaacctgcctatctttttccatttgctgtcgtgtttgcaaagaatccagtttatatttttcagtctcatttaacaattctactatgcgactgtgtttttcctctagctgtttctgcagctctttcagtaggtcctctgagggcaagggtggccgagactgtccagtaccatcactgctctgcagctgtgcgtgcaattcccgctccctatctagggtactactcatttcccgaattcgaactttctcagattcaagaagtacctgaagctctaagtttcgaccttgttcttctgacaactgggcatcatatagcattctctgtgattctattttttgctgggattcgttcagtagttgtttctgttgttccaaaagtagatttagctgaagattcctttgtttctgactctcaagtgaaaacttcagatcctcaagttcttctttatcccgttcttcactgcgtcccaacttggctttctctttctccaaagcccactggagctctcttgattttttctgttcacttgctaatgtgtcattaagcaaatgtacttcatctgtcttatctttaacttccaacctgaaagcctccaattcttttaggtgtttatgctgtgccttgagtgttgtttctagttccaatttagtttgtgcaagctcactcttcagttcagcaaccaccattttctcagaactcagctgctcctgcagttccgttgctctgtctttcatactgctgagctccacttgcatctccagcatttgagactgcttctgctgtatattatattccaagagttcttggcttggtttctcactctcttgttctcttttcagagtaattttcctaccattcatttgtgcatgcagtgcctgaatttcagataacaaactccttctatctgctttctggaggcattccatagctgcttgatattcaacaccctgttcttgtattctctgttccaaacagtttagtaaaccaactgcatctgtagtacctagagctgtcagctccgtccgaaatgctgctagtaaaacactacgctcttctaagaaaacttgttgaagggcaagcagtagttcacctcgccagtctgagaagctctcatgagattgagaactatcataaacctcggcttctctttgcagttgcatctttgtaattaaatcctttagagatgagattgtattgatgtaagcttttctctcttctagccaaggttctgaaacctgctgaatagaatggtcctctccatcactatagggagactcagtgagagaaagcacctgcatgccttcattatggacagctctcagtaatccctttattttctttggaaaggaatctgttgcactttcactttcttctcctcggccttctgatgctatgtcaaatccctgactgtgtgtaagataaattccctgaccccagtctgatccagaatcactggagcatatttctctagtctggtaagcatcagaatgtgctagctcaggaattgaggatccctctttacttctcagacactgtatcactgccttcaaggtaccacattcctctttcagtaactgaacggcaacatagtgttccctctttaaggtttcagtttctgaaatatgtctggattccatgtccaaaatttcagcagcatgtagttcttgcatcttctcaattttttcagtaaactgactgattatttcagtaacttcttctgaggaacattcactctgtaaattaatttgtattcctgcatttttaacaagaatttgtggagtctgattgctgctactgatcttcagagtcccatctgtctgggatgcaatgctcttactcagttttataggaagtggctcaaacatgcaggcctttttgctttcttgtacctcagtctcatcttctttttctaaaatggacaatttctcttttgcctctgcgaggtgatccctaacttggcttaagtctttctgaagagatgtcatatttgtttcttttaccaaaagctcttcttgaagtttttcagccttttctttataactggcaagttctgctttggtagccactgattcagctctaagagcctcgagttcattaaaaaatccactttcttcattgctatgaaatagctcagtagttgtcttgagaacttcaacatcttgagggcttcttttcttttctttctctctctgttttttctcattgccctccaatagcttctgtagttctagcagcttcttttctttttctaaaacatttttttctgcaatttctacttgttctttttctaaaatcaaactagtatgcatttcaacaacctggctttctaattctgatattctcaaggttaatgctgatatatctgaccccaactcatcttctcttagttgatttaaattctgaatatttgttctttcaggttctgatgaaattgtttgattatcttgacagaattttgcatattcctgaactgcctcaagttggatttgactgacaagagcagcagccactttttcttcaactattttctgtaggtttacaatcttcttttgaagcatttctgtttcaaactggccttgttcttgcatgtcttttatttgtttataacactgggtaagttctaagtcctttgcactaacagtgctctcaagttgtagcaaccttgtttccaaattaattatggaacctttgccattttcttcaaaagatttgaagtatgtctgattttctagggatttaagagcatcctctgtaaggactacttctagttcaggtttgtctttgctcagatgatctatagccacgttaacactattctctggtatgctttgaatcttttccacactttcacgttctctctttaagctgaataattcctgtgttagctgattcattttaaaattggtttctttaagtacatttttcatgaaggtcatttcttcattagcggtttctacttgctgttccaaggccagcttttcagctataaccacatccaattgatgttttaaactgtctgcttcttctgagagggaatgagcattcattgatgtcttctgtccaatatttgccaattcctgttgaagtttttcaatcacttcattgagctgctctatttcttcttctctatttctcttcacacattcttgatcactcatcaaacattctatttgggtttcaagatcccttatcagttcatttttttcttcaataaccttgttatctgttgtaattttaagttgctgctggagtttcgtaacttgttcatttaattggtcaatttctacctctttttcctgtattatttgagcaaatttcccaaatagcacatgttggtcttgagtagacatggcatcagattcctttatggcaagtcccagtttctccatgtcatccttaaataatttgttttcctgttcaagttcttgtaggcgggtagtagattcctttttctgtatttctaattgcatatgtaattgttgaacttcttcattcttattttccagttcttctctaaactgttctaattgctcttctaagtttgtaatctctttttcctttctgtctatggcatctcgttcagcctgcaattgtacttctagggacaattctggtttagcttctacagctccaaagtgttttcggtcctctaccttttgaaaagtatctgcactcacaagaagcgcctgctccagttctcttactctgaactccagtttctctatttcttcattcctttcttgtatatccctttgaagctgctctttagagagcaaaagctcactgcatttgtctgttttttctttcagatgatttgctaactgttcaacctctctagtttgatgttcactgataggctggaatcgaggaacaaccttaagttgctgttctagtttctgtatttcctgttggaatacatctctctcatgttctctgtcaatggcttgctcatctaaaaattttctcattttttctaactgcttttccaatgcttggttttgctgtcttaaatccattagttcagtatttttttcttgttccagctctataaacctactgacttgttcttccacatctatttctagagctttcacttgtttttgaaggtcatcacgtactttttcagcttgacattgtacttctagtttttccttcattaatttttctgtctcctgtagtaattctgctcctggtgctgcatcgactgcagcatctactagtcgttgttcaactgggcctgcctctgctttcatagcttccttttgtctggacagtaattctctttcttcttggatctgctgttgctctgcctccaattcttgcaacctgttacttgcacataacaactcctgctcaagacgatctattatatcagttttttcctgaatttgcctttcaaaaagagttttttcatctgcatagccatcaatgacgccctcagccttactgagctccacagctagctgttctctggccctggactcctcatgaaggcgctctcgaagttcctcttggcacttaagggactctgttgcttcttgtttctgtctaaatgactcacgcatcaactctgtctgtgtcactttcgcatgttcaagtgaataaggaggggtaggcagtgaaattttagaaataagctttaatatatgcccgtttcttttatgaataaaatggaaaatagaagtattaacaattactgagttattttcatccaaatgttcacaaagaggaaaaggatgtggtaaaggcacgcgagattcaacctcataaatgtcttcatcttgctcttctaaccacgagccactgactttgacagttgccaaataggtgctataagaatccatcccagaagatacagctgccgagattcctaatttgctttatcaattttctaatacattaaaaagttctttttagtttatcaagatctaccatagcagtataaaaagtttcttttttagcactatcaaataaatgttataaaattaattcatacaactgcacaataaaaggaaggggaaagtccaggaaaaaaactacaaatctaaaaaaacttaggtctctatcaatcttgatgccccctcaaaaaaacccaaaccaaaacaaaaaccaaaaaaaatcaaaaaacaaaaataaaagcaagcaaacaaaaacaccttttaaactagcataattaagtccttgaagagaagaataaaaatataaacatctaattagacgagcaataaaactgcttttaatatcagcgatgtctgtagtaataagtaagccttcaaagcagaacctggcagggaaggtcaagtttgaaatctccatagcagcagtcttgagaaatgcagttgtaacattatttctcttgctcttgctgcttcactctattcaaaaggaaaagctcttct

SEQ ID NO: 14136 - RNA, 15964 nt, Homo sapiens
  source 1..15964: mol_type = other RNA
gctgggattacaggcatgagccaccgcacctggccttccctgcttcctctctagaatccaattagggatgtttgttactactcatattgattaaaacagttaacaaacttttttctttttaaaatgtgagatcagtgaactctggttttaagataatctgaaacaaggtccttgggagtaataaaattggtcacattctgtaaagcacattctgtttaggaatcaacttatctcaaattgtaactcggggcctaactatatgagatggctgaaaaaataccacatcgtctgttttcactaggtgatgccaaaatattttgctttatgtatattacagttctttttaaaacactggaagactcatgttaaactctaattgtgaaggcagaatctctgctaatttttcagattaaaattctctttgaaaaaatacagtctgtattcatgaattgtaaaatatgtgcttcagtgagcagagttagggaatccaggaacttgggtggggaaaaattacatctttatttgcactaataatttctaactgcaatttagtatttatttcaattatgaatttgggcagcattttattagcagtatccatgattttgtcaatagaaatctcagatattttcatattacagatgttacagatttcttgaagtatctagttacgaccccgagataaggctagtctaatgtttagtgaatagttttagacttcttaacagatttcatttttaatcacagactaattaattattgagatgcataaacaagtgtgattgcagaggcctactatcataaggaggcgtggtggtcaaacaatggcactgaactcagcttgatcagatcatttgtccatctgtttttttctccactgtctcttagagcagaatagccttgaatggcaagccatgctagctgaaaaaggtttttacccacaacctgccccttcaactaactgctttagagtacgtttgctatttttagaattcctcttattggaacccagcttctaatgtggaaaatttaagtatagttggctccttttatttgtgggttctgtatcctctgattcaaccaactgcaggttcaaaatactaaaaataaaaccccacaataaaaaaatacagtattagcaactatttacataatgttcacattgtattaggtatcaaataatctggagatgatttgaagtacacaggaggatgtatgtagactatctgcaaatagcacattgttttataagagacttaagcattcgcggactgtaatatccaagggggatcctggaactaatcccccacacatgccgagggatgactgaaattagaaatgttcaagcatgtacaactttctaccatgcctgtttgtgttggtataaatcatggaacatcaaataataagacaaaatcctccaggtgtaagcatcaaatactagtcctcttgctgttttagtgagttgccatgttattgaggaggactccagatgagaaataacattgcgatctgtattatctctgtgagagcctcccagtctgaatttggcttggacaacagggatactgtttaattcggctgcaatgtgattaagatcttttgagttaatgatttcttcatctttttagtgggccatggatttgtgagaacacatctttggaaacaagtaacactaactgtaatatagtaaatactgattaatcatgaaataccaatatagcttttaaaaaacactatgtagatgtaaagttgatacaaagacacatggaaaactttcaacagtattaactctaagattaggacaactttctctgaatctctcactcctacatatttgacataagtaatgagatgctatgtaccaagaactatggctcagttaaaaatgaagaaggttcaaatacagtgtggtgaaaatggtgaagtcatttttatttcagtacttgacaaaataccccataaaattcaaaacttctaccattatacaaaaataggtctctacaagtgatattatctgtcttcatcaccagtagaatatattaggcaaaacatgtaacttcagtagccttataagaaaagtgcaggacacctcgagctacacattcagcagtattgtaatgcgtaaaagtttaatcttttcacccatttgataaatacacaaggtttataatttaatgttttaaattagcattccacaaatatacaggtaattcaataattattgtgcatgaatacatacacaatgcttatatatacaaattccagtttgttttcatgtgctggcaagggatttgtatacaatcataagctgtgttcatattggtcccattgaatattcacaatacaaaagcacaaaagaaccattgatttacaaaaggaaatctatttaaaatcacttcaattaatgatgtttcaaaggattatcttctcatgccagcatgaaattgagtagttgaacctatgagagaaaaacaggaaattcaactgatttcaaattacattgctacctgtatcagacccaccagagttcacacaaaggaaattattattattctccatttttttaaagccctttttttccttaaaatgtcctcttcatacttaaactgagtctctccccactacccccaaggtggagtgttactctgttgcccaggctggaattcagtggtgtgatcttggctcactgcaacccccgcctcctgggttcaagtgattctcctgcctcagcctcctgagtagctgggactatccacacatgccaccatgtccagcaaatttttgtatttttagtggagacggggtttcaccatgttggccaggctagtctcgaactggttggtcttgaactcctgacctagtgatccgcctgcctcggccgcccaaagtgctgggattacaggcatgagccaccgcgcccagcccatatacttaagctgacttttaagagattttgaatatatatgtaaaaatcaccatgactggctctatggcaaggtaggtgagactaatatttagagtttttttaaagtgctctcaaagttggatgttctatacctcatacatttttgaaaaatcttttggtcttcaaaatctgggtcttgtgaaatttggatgctcaaaacaaaacaagcctaggcaaaccaacaaactcagctatgataataaaagtttcctattactacaagatgcttgggtgtaaacaaatgatttcttgaaggaagagataaactactcaatgattcaaagtctctgaatcaggagtgaactgaagtgagatagggaaaagaggttttccttccatgaacagggaatccacctttattttaaagtatgacttgttttttgtttttgaacaaagaaaaaataatccttacaaagtattttaaatgggatagtttttttcgatgatacataaaagcacaatatagtagcagggataatggttacattaagtgcttaaagtaagtgcttcctccttaactccacccgatttgcatgccttaccactttcttttttttttttttttctttgagacagggtctcgctctgctgcccaggctggagtgctgcggcacggccttaccactttctgccatgcgctacttaggaatacgttctccagttaggctctgtagactcagagtaccttgcacactggtgctcattgtgcattttgtgtcatcagtccgctgaatgaacatagtaggaaatcatttttgggaggagtgggatctggggtgataaatcatattttcacttaaattatttaaagtcagtttctctgctggttacaagagtttaagctttggctaacttaataattagctcatgcactaaactggaagctttgattatcctaatgagtgtgaaagaatttcaaagaaaggggagctgtgggtctcgcactgtggtgctgccaagatgtggttaaactcagagcacctgactgtatagttccaagtcgtctttgcagtgcctctagccgagtgatataatctgttagggctctgtcaggatcgtaattctgaagctgagaacatgctaaagaaccaggattgaaatcagctggagtgcctgggtacctattctgaaatggtaaaggggacctaatatagtccagatctgatcttgagcgatacgtagtatgtcttggttctccatataactccagcccaccagaagaatgataaaatgagtcagtcttttctgcaccttgattcagtccaaagccatctctgttaatattgatggaaacagaacctgtgactcgatgccaccgtcgaaccaaaaatttcattctggaaattgcaatggatactctgacggccgaccgaaacctggtgaagccctttgggcgattggtgatcacctctagatccgtgaaagctggctgcccccccatccgggcaagcagggccaaggtggcatcttcacattcctggaacccacccagtaacagcagcaggtatttcttctggtaaatgagagcctttcgaaaactttctgccctcaagtatttaccataaattctctttaaagtgacatgttcagaatcagggctcagagtttgaagtaaagagtcatttcttagttcagctttcagtttgtatacttcagcctctgcccttttcaaagatttctggagagtcaatttttctctgttccatacttctttttcagaggcaatgatggcttcaatgttggcaccaccattcaatgaaaacctggaagaattatctctaccagctcctgtctgtcgataccacctgatctgctcttccagcttcataaccatgttccttaagtcattcttctcttcagtcagttgactgatatgccctgtcagctcagcattttgtctcagtagtctttcagtcaatgagccacaagaagtacttggggacaccaagctgggctcttcaccttgctggccagttaatttctgtagttgtaaaataatttcatcaatattttcctgaacccaaatgaaatcttcatcatctgctgtttcaaactgtagtctctcagaggctttctggggtagaacctgtagttttgaagctacacattgaagcttttgtctgatcatttctaattcatgattacagccggttcctcctccattcatttcaatcaatttagcgtagtttgattcttttgtttctccttctattttctgttgaagaacccaatttctagttctatcactggttaagctccacgtggttggctcattaaggttctgatacagaattcttctactttctcgtttttcttctcgttctagttcttgcttctggaattcctgcatgattccttgtagtcgctgtccttcaaggtctaacttataaacttgttgtcttttctcttccagctggcgctgaagatcttccactttggactggagctcatgcatttttttctgtccctcagtgttggcctcctgttctgtctgcagtgttttcctgtgaacctgcctatctttttccatttgctgtcgtgtttgcaaagaatccagtttatatttttcagtctcatttaacaattctactatgcgactgtgtttttcctctagctgtttctgcagctctttcagtaggtcctctgagggcaagggtggccgagactgtccagtaccatcactgctctgcagctgtgcgtgcaattcccgctccctatctagggtactactcatttcccgaattcgaactttctcagattcaagaagtacctgaagctctaagtttcgaccttgttcttctgacaactgggcatcatatagcattctctgtgattctattttttgctgggattcgttcagtagttgtttctgttgttccaaaagtagatttagctgaagattcctttgtttctgactctcaagtgaaaacttcagatcctcaagttcttctttatcccgttcttcactgcgtcccaacttggctttctctttctccaaagcccactggagctctcttgattttttctgttcacttgctaatgtgtcattaagcaaatgtacttcatctgtcttatctttaacttccaacctgaaagcctccaattcttttaggtgtttatgctgtgccttgagtgttgtttctagttccaatttagtttgtgcaagctcactcttcagttcagcaaccaccattttctcagaactcagctgctcctgcagttccgttgctctgtctttcatactgctgagctccacttgcatctccagcatttgagactgcttctgctgtatattatattccaagagttcttggcttggtttctcactctcttgttctcttttcagagtaattttcctaccattcatttgtgcatgcagtgcctgaatttcagataacaaactccttctatctgctttctggaggcattccatagctgcttgatattcaacaccctgttcttgtattctctgttccaaacagtttagtaaaccaactgcatctgtagtacctagagctgtcagctccgtccgaaatgctgctagtaaaacactacgctcttctaagaaaacttgttgaagggcaagcagtagttcacctcgccagtctgagaagctctcatgagattgagaactatcataaacctcggcttctctttgcagttgcatctttgtaattaaatcctttagagatgagattgtattgatgtaagcttttctctcttctagccaaggttctgaaacctgctgaatagaatggtcctctccatcactatagggagactcagtgagagaaagcacctgcatgccttcattatggacagctctcagtaatccctttattttctttggaaaggaatctgttgcactttcactttcttctcctcggccttctgatgctatgtcaaatccctgactgtgtgtaagataaattccctgaccccagtctgatccagaatcactggagcatatttctctagtctggtaagcatcagaatgtgctagctcaggaattgaggatccctctttacttctcagacactgtatcactgccttcaaggtaccacattcctctttcagtaactgaacggcaacatagtgttccctctttaaggtttcagtttctgaaatatgtctggattccatgtccaaaatttcagcagcatgtagttcttgcatcttctcaattttttcagtaaactgactgattatttcagtaacttcttctgaggaacattcactctgtaaattaatttgtattcctgcatttttaacaagaatttgtggagtctgattgctgctactgatcttcagagtcccatctgtctgggatgcaatgctcttactcagttttataggaagtggctcaaacatgcaggcctttttgctttcttgtacctcagtctcatcttctttttctaaaatggacaatttctcttttgcctctgcgaggtgatccctaacttggcttaagtctttctgaagagatgtcatatttgtttcttttaccaaaagctcttcttgaagtttttcagccttttctttataactggcaagttctgctttggtagccactgattcagctctaagagcctcgagttcattaaaaaatccactttcttcattgctatgaaatagctcagtagttgtcttgagaacttcaacatcttgagggcttcttttcttttctttctctctctgttttttctcattgccctccaatagcttctgtagttctagcagcttcttttctttttctaaaacatttttttctgcaatttctacttgttctttttctaaaatcaaactagtatgcatttcaacaacctggctttctaattctgatattctcaaggttaatgctgatatatctgaccccaactcatcttctcttagttgatttaaattctgaatatttgttctttcaggttctgatgaaattgtttgattatcttgacagaattttgcatattcctgaactgcctcaagttggatttgactgacaagagcagcagccactttttcttcaactattttctgtaggtttacaatcttcttttgaagcatttctgtttcaaactggccttgttcttgcatgtcttttatttgtttataacactgggtaagttctaagtcctttgcactaacagtgctctcaagttgtagcaaccttgtttccaaattaattatggaacctttgccattttcttcaaaagatttgaagtatgtctgattttctagggatttaagagcatcctctgtaaggactacttctagttcaggtttgtctttgctcagatgatctatagccacgttaacactattctctggtatgctttgaatcttttccacactttcacgttctctctttaagctgaataattcctgtgttagctgattcattttaaaattggtttctttaagtacatttttcatgaaggtcatttcttcattagcggtttctacttgctgttccaaggccagcttttcagctataaccacatccaattgatgttttaaactgtctgcttcttctgagagggaatgagcattcattgatgtcttctgtccaatatttgccaattcctgttgaagtttttcaatcacttcattgagctgctctatttcttcttctctatttctcttcacacattcttgatcactcatcaaacattctatttgggtttcaagatcccttatcagttcatttttttcttcaataaccttgttatctgttgtaattttaagttgctgctggagtttcgtaacttgttcatttaattggtcaatttctacctctttttcctgtattatttgagcaaatttcccaaatagcacatgttggtcttgagtagacatggcatcagattcctttatggcaagtcccagtttctccatgtcatccttaaataatttgttttcctgttcaagttcttgtaggcgggtagtagattcctttttctgtatttctaattgcatatgtaattgttgaacttcttcattcttattttccagttcttctctaaactgttctaattgctcttctaagtttgtaatctctttttcctttctgtctatggcatctcgttcagcctgcaattgtacttctagggacaattctggtttagcttctacagctccaaagtgttttcggtcctctaccttttgaaaagtatctgcactcacaagaagcgcctgctccagttctcttactctgaactccagtttctctatttcttcattcctttcttgtatatccctttgaagctgctctttagagagcaaaagctcactgcatttgtctgttttttctttcagatgatttgctaactgttcaacctctctagtttgatgttcactgataggctggaatcgaggaacaaccttaagttgctgttctagtttctgtatttcctgttggaatacatctctctcatgttctctgtcaatggcttgctcatctaaaaattttctcattttttctaactgcttttccaatgcttggttttgctgtcttaaatccattagttcagtatttttttcttgttccagctctataaacctactgacttgttcttccacatctatttctagagctttcacttgtttttgaaggtcatcacgtactttttcagcttgacattgtacttctagtttttccttcattaatttttctgtctcctgtagtaattgttgttcaactgggcctgcctctgctttcatagcttccttttgtctggacagtaattctctttcttcttggatctgctgttgctctgcctccaattcttgcaacctgttacttgcacataacaactcctgctcaagacgatctattatatcagttttttcctgaatttgcctttcaaaaagagttttttcatctgcatagccatcaatgacgccctcagccttactgagctccacagctagctgttctctggccctggactcctcatgaaggcgctctcgaagttcctcttggcacttaagggactctgttgcttcttgtttctgtctaaatgactcacgcatcaactctgtctgtgtcactttcgcatgttcaagctgactgctagtttcacttatggcttctaggagtttttcaactgctgcttgtagtcgagagctaatgttcagcataagttcttcattttcagggtctatttcagttccagcaaaaccactcctcacaagtcgttgtgacagctctgttccttcctcagttacttttgaccacatgttaatgtcatttcttggcatatcacttccagaataagagggaatggattcatctgtaactcttgtatgttcctcatggacacatgactttacagatgcctctgcttctgacctccaaattaggctggcagatgactggcttttactagatctatctagaatcccaaggacatggcgaccaattgtttcttcaacagctgctgttgtctttacaacttctaagaggatcttcaaaagtctattattagctttctggagtgcatacactgtctttcttgtttgagttccatactgactgcgttccatactgatgatccaatggggaagccaaaatcttaggggccaaattcctccatgcaagctttcattagacaaaatctcaggaggcacatcttcaggttttctgtctaattccttttctttaaatgtttgttcttcaacttctccttggttttcatttccattctgtgtttgcgtactgctgttgcgcagctcacaacacagcttctctcttccagctaaagacagctgctttagtgcttccagctcctctaaaagcaccctctctctctctgaaaccaggttttcattatctatggaggatctctgggctaattgtctattaagtctcttaatctcttcttgtagctgttcctggtcttctcgctgtctctccatttgccgcatatgtgcttgccttaacaattccgttgcctgttgatgttcttggtattgtcgtacaagttcctgtctcatatcttccaactgttcttcattcaacattagttgtctagaagcatccatgcttgacactgaaatctcatcatgaatagactgtctaactataaatgttttatctttggagaacatttcttctgaaatagtcagcacacagtcctttgattctggtatatcatggggatcactatttgataataaaatttcctttccatgttctcctaactctttactaagtggtttaaattcttctttaaatttcacatccactgtctcaaaagtctgaaaaccaatttgatcctgtgataatttcatttcattaaaataatgttgttcttgctgacacacagcatgtgcttgctttgatgatgcagtattttcttttcccccagatattctagacagttcagtttgttgagcaaatgctatactcattgacacaataaccttagctacttcttcttctaattgttcttggtattgtttttcaagcaacttaacgatatttgtttcctctttcactccaaattcaccagaaaactctattgtaccatcaatattctttttcacacaacttccagggtacattgttctctgtgcatcagattctgtaattaccaccgaatcaacaggtaagcttggcggaaccgtggactcactaacagcttgaagcctcttctgtaaacagtggatctctgcctcatagttttgttcagtttctttcaactgttgctgcaaagaggatatgaggctttctaattcttgaacttgttcttcaagtttagttttttcaagatcttgcagagaagataacttgcttttatgattgacatcaatgtcttccaaattggtcatctgagaatggattgataaaaactctgtttcctcttttggaaggttttcttctccaaattcaagtttcataccatctgtctgctgtccccagatcttgcttagtcgtgtttgaagtaccaagagtttgttgtattcttctgttactttgttgagaagagtgtgcatattttcttgaaagtcttgaacttcatatctataatcttgtaattctggatcttcattttcagaaatgtaatcaccagaattctctttgtcttctgcatttacttcacattttaaagcaggagtataatattcaccaaggacactgcataaagtctgtaaaaaataagaacattcttcagacactgccttttgaagttttccaatgagcagatgtaaaggctttccttcatcacctgtttcttgtgttttcatagtctgtagttctaactggtgtattttctgaagttccttgatcttttcctcttgagcaaaaataagctcttctttaagactgcaaagagctttatctttttcattttccatatattcacgaacctgatccacatgagttgaataaaccagagagaggcaaatgcgttgggcttccatctgtagccttaaatcattctgttctgatttaagtacattgagttctttctgaagtttatcattttcacttggttgagttgctctaagtgatgattcctttgttacagatggtaagtgatccaaaatcaactgttcttgcttactttcttctccaacagtcatattttcaaaagaaactttatcttccaccattatttttgattcttcaccaaaacttttatttactttagaaactgatccttcagcacccctgcttgtcatggtcacaactccatctaataaagagcttacttgagtatcacatgactgtacattttctgccctgttgtggttaataatgatttctagctctctacatctcaatgaaacttgttctttctcttgctttaaagatttaacttcttcatttagaaaactaatctcaccatgtttctgtttcaattgttcagaaagatcagacagtctctgtgacagctctaatttctctcgcttggttacctcaagtttttccatgagttctgttgtatccttttcaacaacctcacccatttccaatgtttctgctacaaaagttttgtcttcatcaaagacagaacttttcattttcactgtagttggatttattctttgcaaatgaagctcttcattaagtgctttaagtttacttttatactctaattcctgtttatttttactgtcttctaaatcatcttttactttgagaaggcaagcatactcctcttgtaactcttgatagttaacttcaaagtttttttcagcaaatgaaaaagtgttcctttgcttttcaatctcttcatttagctgaatacattgttgtttgaggtcctcattttcctctataagtatttctatttctttttcccacacagagtctttggatttggacttaatggagtctaagaaaatcaatctttcttcttggctaacaggagtatgtattttcaacatgtcttcaagggttttcttttcatctttaagaatgctattctctgcttcaagttgtgcaaatttttcttgaagatcattctctttttccttcatctgtttttctaacaattctgttttaagttgtaattcttgaacttcttgttcaagtgtacccttttctttttcttcttgtctgagtatttcaatttctttttgaagttcattgatttgaagagtcatttcttctgactttgaatttacaagagactgctgtaaatcttttagctttgaaatttccaaaattaattgattctgcttagttatcaaattgtccttttcaaactgcatggtttctatcttttgactcatttcattctgtaaaccatctatctgctgtttatagtgaatgcctaaattatctttaagtttttcaatatttattcgatgttcaatttctaaatcttccttcagtttggaaagctcttcttcgtgactaaatagaagctgtgttctcagcctctctaattcagcttcttgtgattcagccattctgtctaacacagcattcttttctttttctaacatttcaagttttatcttgtaatttgtaacttctgcttcatgttttaattctagttcctttctggattcagatgcagaaacaatctcagctttcaaatcttccactgtactaagggacttatgtgcttcattaagtttactttcttgttcagctattgtctgtctagctctctgaatctgttcccttgaaaagctcaattcttcaacaaggtcttcaagctgtctctgtagagcacacttttcttctaaaattagtcctagttcttccttgagtttttccttttgagagttagtatcttgcaattttatattcagttcatttattgccacattcattaactttatctgatcttcattaactgtaatatttgaatatgaccttaaagcattctccatttctcccttatgccgtgttttcatttcctccatctgtgccatgtgttgtcttattaattcttgtttcatttgcactatctgctgcccatacatctcatccagctctgcccggagttgttctaactttctttgtgtttcttgttccattcgttgtactatatcagtttcgaactggctgtctttatgatttctcttctgaagttcttcgactgtccccattaactgttttatttcttcagaagactgtctttctttttgcttagaattagtcagctctaatttcatgttttttatttcttggttcttttgcacaatctgttcttgtaattctcctagtaatttatcagcagttgttaatttatcctttagctcaagagttttcttttcttcttctattatttttgtgtttaattcttcaatgattgtctccttttcctgtatttcttctttatttgagttttctacttttttatcttgttccatttcatatactttaattttctcttgcaagaaactaatttgcattgtgaagtcttctttctttttctgataatcttctaataagtggtcttgttcttcaagctgctgttgatgagtgaggatctgttgtttggcttgtagtaagtctgcagctgtgctactatgagtgctgtttctcagagtttcactagcctgtaattgctgaaattgaatctgtaatttttgactctgttctgtcaactctaaaaattctctcattgtctcatccttttctcttcttgcttgttgtaaattagcagtgagctgggttataatgccatctctttgtttaatggcagcttcaaattcttgtaactgctgcagtccttcagtcccataggtaaccctcatttcttccagctctctgtttagctcttcaatctcatgctgcttcccagccaactcactttccatcatctctagatgagtcggactgtcttgtgctccttgttcagaataagaatcatcaacaccaaattcttcttcccttaataaatttgtaggctttcctgttctcatcacaaaactgcaaccatttacctctgaactgcagtcatctgctgtggttgaaatttcactttccagttccacagagaagccctgctcatgactggttatttctccactatgtagagttctcattattgtagattcaggaatcacagttgattctactctctgagaactatttatgtacatttcattacactgtgattgatcaatattcaaatcatggtgtgctgacacatcatgtttactgcttgacgtttttctcttttttttctgcttcttggaaggactctgcccatccgactgagcttttctttgtcgaaactgggcaagcttggctttgccggcctccagcttcttctgtctctcctcgtcctccatggcctctgcaaggaaggcaggggaaaacaggggttgaggggtggttggggatagaaaggaaaggtcgatttggacggaggtgggacggcaagctccacggcctagagagccgattcggtccggcgctcccccgcccgaagtggaagcagtctccgcgctcactggcggatcgtcctcagccgcacgggaagcgccgtcaccgccgccgccgccgccatcttcgtctccacgta

SEQ ID NO: 14137 - RNA, 15727 nt, Homo sapiens
  source 1..15727: mol_type = other RNA
gctgggattacaggcatgagccaccgcacctggccttccctgcttcctctctagaatccaattagggatgtttgttactactcatattgattaaaacagttaacaaacttttttctttttaaaatgtgagatcagtgaactctggttttaagataatctgaaacaaggtccttgggagtaataaaattggtcacattctgtaaagcacattctgtttaggaatcaacttatctcaaattgtaactcggggcctaactatatgagatggctgaaaaaataccacatcgtctgttttcactaggtgatgccaaaatattttgctttatgtatattacagttctttttaaaacactggaagactcatgttaaactctaattgtgaaggcagaatctctgctaatttttcagattaaaattctctttgaaaaaatacagtctgtattcatgaattgtaaaatatgtgcttcagtgagcagagttagggaatccaggaacttgggtggggaaaaattacatctttatttgcactaataatttctaactgcaatttagtatttatttcaattatgaatttgggcagcattttattagcagtatccatgattttgtcaatagaaatctcagatattttcatattacagatgttacagatttcttgaagtatctagttacgaccccgagataaggctagtctaatgtttagtgaatagttttagacttcttaacagatttcatttttaatcacagactaattaattattgagatgcataaacaagtgtgattgcagaggcctactatcataaggaggcgtggtggtcaaacaatggcactgaactcagcttgatcagatcatttgtccatctgtttttttctccactgtctcttagagcagaatagccttgaatggcaagccatgctagctgaaaaaggtttttacccacaacctgccccttcaactaactgctttagagtacgtttgctatttttagaattcctcttattggaacccagcttctaatgtggaaaatttaagtatagttggctccttttatttgtgggttctgtatcctctgattcaaccaactgcaggttcaaaatactaaaaataaaaccccacaataaaaaaatacagtattagcaactatttacataatgttcacattgtattaggtatcaaataatctggagatgatttgaagtacacaggaggatgtatgtagactatctgcaaatagcacattgttttataagagacttaagcattcgcggactgtaatatccaagggggatcctggaactaatcccccacacatgccgagggatgactgaaattagaaatgttcaagcatgtacaactttctaccatgcctgtttgtgttggtataaatcatggaacatcaaataataagacaaaatcctccaggtgtaagcatcaaatactagtcctcttgctgttttagtgagttgccatgttattgaggaggactccagatgagaaataacattgcgatctgtattatctctgtgagagcctcccagtctgaatttggcttggacaacagggatactgtttaattcggctgcaatgtgattaagatcttttgagttaatgatttcttcatctttttagtgggccatggatttgtgagaacacatctttggaaacaagtaacactaactgtaatatagtaaatactgattaatcatgaaataccaatatagcttttaaaaaacactatgtagatgtaaagttgatacaaagacacatggaaaactttcaacagtattaactctaagattaggacaactttctctgaatctctcactcctacatatttgacataagtaatgagatgctatgtaccaagaactatggctcagttaaaaatgaagaaggttcaaatacagtgtggtgaaaatggtgaagtcatttttatttcagtacttgacaaaataccccataaaattcaaaacttctaccattatacaaaaataggtctctacaagtgatattatctgtcttcatcaccagtagaatatattaggcaaaacatgtaacttcagtagccttataagaaaagtgcaggacacctcgagctacacattcagcagtattgtaatgcgtaaaagtttaatcttttcacccatttgataaatacacaaggtttataatttaatgttttaaattagcattccacaaatatacaggtaattcaataattattgtgcatgaatacatacacaatgcttatatatacaaattccagtttgttttcatgtgctggcaagggatttgtatacaatcataagctgtgttcatattggtcccattgaatattcacaatacaaaagcacaaaagaaccattgatttacaaaaggaaatctatttaaaatcacttcaattaatgatgtttcaaaggattatcttctcatgccagcatgaaattgagtagttgaacctatgagagaaaaacaggaaattcaactgatttcaaattacattgctacctgtatcagacccaccagagttcacacaaaggaaattattattattctccatttttttaaagccctttttttccttaaaatgtcctcttcatacttaaactgagtctctccccactacccccaaggtggagtgttactctgttgcccaggctggaattcagtggtgtgatcttggctcactgcaacccccgcctcctgggttcaagtgattctcctgcctcagcctcctgagtagctgggactatccacacatgccaccatgtccagcaaatttttgtatttttagtggagacggggtttcaccatgttggccaggctagtctcgaactggttggtcttgaactcctgacctagtgatccgcctgcctcggccgcccaaagtgctgggattacaggcatgagccaccgcgcccagcccatatacttaagctgacttttaagagattttgaatatatatgtaaaaatcaccatgactggctctatggcaaggtaggtgagactaatatttagagtttttttaaagtgctctcaaagttggatgttctatacctcatacatttttgaaaaatcttttggtcttcaaaatctgggtcttgtgaaatttggatgctcaaaacaaaacaagcctaggcaaaccaacaaactcagctatgataataaaagtttcctattactacaagatgcttgggtgtaaacaaatgatttcttgaaggaagagataaactactcaatgattcaaagtctctgaatcaggagtgaactgaagtgagatagggaaaagaggttttccttccatgaacagggaatccacctttattttaaagtatgacttgttttttgtttttgaacaaagaaaaaataatccttacaaagtattttaaatgggatagtttttttcgatgatacataaaagcacaatatagtagcagggataatggttacattaagtgcttaaagtaagtgcttcctccttaactccacccgatttgcatgccttaccactttcttttttttttttttttctttgagacagggtctcgctctgctgcccaggctggagtgctgcggcacggccttaccactttctgccatgcgctacttaggaatacgttctccagttaggctctgtagactcagagtaccttgcacactggtgctcattgtgcattttgtgtcatcagtccgctgaatgaacatagtaggaaatcatttttgggaggagtgggatctggggtgataaatcatattttcacttaaattatttaaagtcagtttctctgctggttacaagagtttaagctttggctaacttaataattagctcatgcactaaactggaagctttgattatcctaatgagtgtgaaagaatttcaaagaaaggggagctgtgggtctcgcactgtggtgctgccaagatgtggttaaactcagagcacctgactgtatagttccaagtcgtctttgcagtgcctctagccgagtgatataatctgttagggctctgtcaggatcgtaattctgaagctgagaacatgctaaagaaccaggattgaaatcagctggagtgcctgggtacctattctgaaatggtaaaggggacctaatatagtccagatctgatcttgagcgatacgtagtatgtcttggttctccatataactccagcccaccagaagaatgataaaatgagtcagtcttttctgcaccttgattcagtccaaagccatctctgttaatattgatggaaacagaacctgtgactcgatgccaccgtcgaaccaaaaatttcattctggaaattgcaatggatactctgacggccgaccgaaacctggtgaagccctttgggcgattggtgatcacctctagatccgtgaaagctggctgcccccccatccgggcaagcagggccaaggtggcatcttcacattcctggaacccacccagtaacagcagcaggtatttcttctggtaaatgagagcctttcgaaaactttctgccctcaagtatttaccataaattctctttaaagtgacatgttcagaatcagggctcagagtttgaagtaaagagtcatttcttagttcagctttcagtttgtatacttcagcctctgcccttttcaaagatttctggagagtcaatttttctctgttccatacttctttttcagaggcaatgatggcttcaatgttggcaccaccattcaatgaaaacctggaagaattatctctaccagctcctgtctgtcgataccacctgatctgctcttccagcttcataaccatgttccttaagtcattcttctcttcagtcagttgactgatatgccctgtcagctcagcattttgtctcagtagtctttcagtcaatgagccacaagaagtacttggggacaccaagctgggctcttcaccttgctggccagttaatttctgtagttgtaaaataatttcatcaatattttcctgaacccaaatgaaatcttcatcatctgctgtttcaaactgtagtctctcagaggctttctggggtagaacctgtagttttgaagctacacattgaagcttttgtctgatcatttctaattcatgattacagccggttcctcctccattcatttcaatcaatttagcgtagtttgattcttttgtttctccttctattttctgttgaagaacccaatttctagttctatcactggttaagctccacgtggttggctcattaaggttctgatacagaattcttctactttctcgtttttcttctcgttctagttcttgcttctggaattcctgcatgattccttgtagtcgctgtccttcaaggtctaacttataaacttgttgtcttttctcttccagctggcgctgaagatcttccactttggactggagctcatgcatttttttctgtccctcagtgttggcctcctgttctgtctgcagtgttttcctgtgaacctgcctatctttttccatttgctgtcgtgtttgcaaagaatccagtttatatttttcagtctcatttaacaattctactatgcgactgtgtttttcctctagctgtttctgcagctctttcagtaggtcctctgagggcaagggtggccgagactgtccagtaccatcactgctctgcagctgtgcgtgcaattcccgctccctatctagggtactactcatttcccgaattcgaactttctcagattcaagaagtacctgaagctctaagtttcgaccttgttcttctgacaactgggcatcatatagcattctctgtgattctattttttgctgggattcgttcagtagttgtttctgttgttccaaaagtagatttagctgaagattcctttgtttctgactctcaagtgaaaacttcagatcctcaagttcttctttatcccgttcttcactgcgtcccaacttggctttctctttctccaaagcccactggagctctcttgattttttctgttcacttgctaatgtgtcattaagcaaatgtacttcatctgtcttatctttaacttccaacctgaaagcctccaattcttttaggtgtttatgctgtgccttgagtgttgtttctagttccaatttagtttgtgcaagctcactcttcagttcagcaaccaccattttctcagaactcagctgctcctgcagttccgttgctctgtctttcatactgctgagctccacttgcatctccagcatttgagactgcttctgctgtatattatattccaagagttcttggcttggtttctcactctcttgttctcttttcagagtaattttcctaccattcatttgtgcatgcagtgcctgaatttcagataacaaactccttctatctgctttctggaggcattccatagctgcttgatattcaacaccctgttcttgtattctctgttccaaacagtttagtaaaccaactgcatctgtagtacctagagctgtcagctccgtccgaaatgctgctagtaaaacactacgctcttctaagaaaacttgttgaagggcaagcagtagttcacctcgccagtctgagaagctctcatgagattgagaactatcataaacctcggcttctctttgcagttgcatctttgtaattaaatcctttagagatgagattgtattgatgtaagcttttctctcttctagccaaggttctgaaacctgctgaatagaatggtcctctccatcactatagggagactcagtgagagaaagcacctgcatgccttcattatggacagctctcagtaatccctttattttctttggaaaggaatctgttgcactttcactttcttctcctcggccttctgatgctatgtcaaatccctgactgtgtgtaagataaattccctgaccccagtctgatccagaatcactggagcatatttctctagtctggtaagcatcagaatgtgctagctcaggaattgaggatccctctttacttctcagacactgtatcactgccttcaaggtaccacattcctctttcagtaactgaacggcaacatagtgttccctctttaaggtttcagtttctgaaatatgtctggattccatgtccaaaatttcagcagcatgtagttcttgcatcttctcaattttttcagtaaactgactgattatttcagtaacttcttctgaggaacattcactctgtaaattaatttgtattcctgcatttttaacaagaatttgtggagtctgattgctgctactgatcttcagagtcccatctgtctgggatgcaatgctcttactcagttttataggaagtggctcaaacatgcaggcctttttgctttcttgtacctcagtctcatcttctttttctaaaatggacaatttctcttttgcctctgcgaggtgatccctaacttggcttaagtctttctgaagagatgtcatatttgtttcttttaccaaaagctcttcttgaagtttttcagccttttctttataactggcaagttctgctttggtagccactgattcagctctaagagcctcgagttcattaaaaaatccactttcttcattgctatgaaatagctcagtagttgtcttgagaacttcaacatcttgagggcttcttttcttttctttctctctctgttttttctcattgccctccaatagcttctgtagttctagcagcttcttttctttttctaaaacatttttttctgcaatttctacttgttctttttctaaaatcaaactagtatgcatttcaacaacctggctttctaattctgatattctcaaggttaatgctgatatatctgaccccaactcatcttctcttagttgatttaaattctgaatatttgttctttcaggttctgatgaaattgtttgattatcttgacagaattttgcatattcctgaactgcctcaagttggatttgactgacaagagcagcagccactttttcttcaactattttctgtaggtttacaatcttcttttgaagcatttctgtttcaaactggccttgttcttgcatgtcttttatttgtttataacactgggtaagttctaagtcctttgcactaacagtgctctcaagttgtagcaaccttgtttccaaattaattatggaacctttgccattttcttcaaaagatttgaagtatgtctgattttctagggatttaagagcatcctctgtaaggactacttctagttcaggtttgtctttgctcagatgatctatagccacgttaacactattctctggtatgctttgaatcttttccacactttcacgttctctctttaagctgaataattcctgtgttagctgattcattttaaaattggtttctttaagtacatttttcatgaaggtcatttcttcattagcggtttctacttgctgttccaaggccagcttttcagctataaccacatccaattgatgttttaaactgtctgcttcttctgagagggaatgagcattcattgatgtcttctgtccaatatttgccaattcctgttgaagtttttcaatcacttcattgagctgctctatttcttcttctctatttctcttcacacattcttgatcactcatcaaacattctatttgggtttcaagatcccttatcagttcatttttttcttcaataaccttgttatctgttgtaattttaagttgctgctggagtttcgtaacttgttcatttaattggtcaatttctacctctttttcctgtattatttgagcaaatttcccaaatagcacatgttggtcttgagtagacatggcatcagattcctttatggcaagtcccagtttctccatgtcatccttaaataatttgttttcctgttcaagttcttgtaggcgggtagtagattcctttttctgtatttctaattgcatatgtaattgttgaacttcttcattcttattttccagttcttctctaaactgttctaattgctcttctaagtttgtaatctctttttcctttctgtctatggcatctcgttcagcctgcaattgtacttctagggacaattctggtttagcttctacagctccaaagtgttttcggtcctctaccttttgaaaagtatctgcactcacaagaagcgcctgctccagttctcttactctgaactccagtttctctatttcttcattcctttcttgtatatccctttgaagctgctctttagagagcaaaagctcactgcatttgtctgttttttctttcagatgatttgctaactgttcaacctctctagtttgatgttcactgataggctggaatcgaggaacaaccttaagttgctgttctagtttctgtatttcctgttggaatacatctctctcatgttctctgtcaatggcttgctcatctaaaaattttctcattttttctaactgcttttccaatgcttggttttgctgtcttaaatccattagttcagtatttttttcttgttccagctctataaacctactgacttgttcttccacatctatttctagagctttcacttgtttttgaaggtcatcacgtactttttcagcttgacattgtacttctagtttttccttcattaatttttctgtctcctgtagtaattgttgttcaactgggcctgcctctgctttcatagcttccttttgtctggacagtaattctctttcttcttggatctgctgttgctctgcctccaattcttgcaacctgttacttgcacataacaactcctgctcaagacgatctattatatcagttttttcctgaatttgcctttcaaaaagagttttttcatctgcatagccatcaatgacgccctcagccttactgagctccacagctagctgttctctggccctggactcctcatgaaggcgctctcgaagttcctcttggcacttaagggactctgttgcttcttgtttctgtctaaatgactcacgcatcaactctgtctgtgtcactttcgcatgttcaagctgactgctagtttcacttatggcttctaggagtttttcaactgctgcttgtagtcgagagctaatgttcagcataagttcttcattttcagggtctatttcagttccagcaaaaccactcctcacaagtcgttgtgacagctctgttccttcctcagttacttttgaccacatgttaatgtcatttcttggcatatcacttccagaataagagggaatggattcatctgtaactcttgtatgttcctcatggacacatgactttacagatgcctctgcttctgacctccaaattaggctggcagatgactggcttttactagatctatctagaatcccaaggacatggcgaccaattgtttcttcaacagctgctgttgtctttacaacttctaagaggatcttcaaaagtctattattagctttctggagtgcatacctttcattagacaaaatctcaggaggcacatcttcaggttttctgtctaattccttttctttaaatgtttgttcttcaacttctccttggttttcatttccattctgggctaattgtctattaagtctcttaatctcttcttgtagctgttcctggtcttctcgctgtctctccatttgccgcatatgtgcttgccttaacaattccgttgcctgttgatgttcttggtattgtcgtacaagttcctgtctcatatcttccaactgttcttcattcaacattagttgtctagaagcatccatgcttgacactgaaatctcatcatgaatagactgtctaactataaatgttttatctttggagaacatttcttctgaaatagtcagcacacagtcctttgattctggtatatcatggggatcactatttgataataaaatttcctttccatgttctcctaactctttactaagtggtttaaattcttctttaaatttcacatccactgtctcaaaagtctgaaaaccaatttgatcctgtgataatttcatttcattaaaataatgttgttcttgctgacacacagcatgtgcttgctttgatgatgcagtattttcttttcccccagatattctagacagttcagtttgttgagcaaatgctatactcattgacacaataaccttagctacttcttcttctaattgttcttggtattgtttttcaagcaacttaacgatatttgtttcctctttcactccaaattcaccagaaaactctattgtaccatcaatattctttttcacacaacttccagggtacattgttctctgtgcatcagattctgtaattaccaccgaatcaacaggtaagcttggcggaaccgtggactcactaacagcttgaagcctcttctgtaaacagtggatctctgcctcatagttttgttcagtttctttcaactgttgctgcaaagaggatatgaggctttctaattcttgaacttgttcttcaagtttagttttttcaagatcttgcagagaagataacttgcttttatgattgacatcaatgtcttccaaattggtcatctgagaatggattgataaaaactctgtttcctcttttggaaggttttcttctccaaattcaagtttcataccatctgtctgctgtccccagatcttgcttagtcgtgtttgaagtaccaagagtttgttgtattcttctgttactttgttgagaagagtgtgcatattttcttgaaagtcttgaacttcatatctataatcttgtaattctggatcttcattttcagaaatgtaatcaccagaattctctttgtcttctgcatttacttcacattttaaagcaggagtataatattcaccaaggacactgcataaagtctgtaaaaaataagaacattcttcagacactgccttttgaagttttccaatgagcagatgtaaaggctttccttcatcacctgtttcttgtgttttcatagtctgtagttctaactggtgtattttctgaagttccttgatcttttcctcttgagcaaaaataagctcttctttaagactgcaaagagctttatctttttcattttccatatattcacgaacctgatccacatgagttgaataaaccagagagaggcaaatgcgttgggcttccatctgtagccttaaatcattctgttctgatttaagtacattgagttctttctgaagtttatcattttcacttggttgagttgctctaagtgatgattcctttgttacagatggtaagtgatccaaaatcaactgttcttgcttactttcttctccaacagtcatattttcaaaagaaactttatcttccaccattatttttgattcttcaccaaaacttttatttactttagaaactgatccttcagcacccctgcttgtcatggtcacaactccatctaataaagagcttacttgagtatcacatgactgtacattttctgccctgttgtggttaataatgatttctagctctctacatctcaatgaaacttgttctttctcttgctttaaagatttaacttcttcatttagaaaactaatctcaccatgtttctgtttcaattgttcagaaagatcagacagtctctgtgacagctctaatttctctcgcttggttacctcaagtttttccatgagttctgttgtatccttttcaacaacctcacccatttccaatgtttctgctacaaaagttttgtcttcatcaaagacagaacttttcattttcactgtagttggatttattctttgcaaatgaagctcttcattaagtgctttaagtttacttttatactctaattcctgtttatttttactgtcttctaaatcatcttttactttgagaaggcaagcatactcctcttgtaactcttgatagttaacttcaaagtttttttcagcaaatgaaaaagtgttcctttgcttttcaatctcttcatttagctgaatacattgttgtttgaggtcctcattttcctctataagtatttctatttctttttcccacacagagtctttggatttggacttaatggagtctaagaaaatcaatctttcttcttggctaacaggagtatgtattttcaacatgtcttcaagggttttcttttcatctttaagaatgctattctctgcttcaagttgtgcaaatttttcttgaagatcattctctttttccttcatctgtttttctaacaattctgttttaagttgtaattcttgaacttcttgttcaagtgtacccttttctttttcttcttgtctgagtatttcaatttctttttgaagttcattgatttgaagagtcatttcttctgactttgaatttacaagagactgctgtaaatcttttagctttgaaatttccaaaattaattgattctgcttagttatcaaattgtccttttcaaactgcatggtttctatcttttgactcatttcattctgtaaaccatctatctgctgtttatagtgaatgcctaaattatctttaagtttttcaatatttattcgatgttcaatttctaaatcttccttcagtttggaaagctcttcttcgtgactaaatagaagctgtgttctcagcctctctaattcagcttcttgtgattcagccattctgtctaacacagcattcttttctttttctaacatttcaagttttatcttgtaatttgtaacttctgcttcatgttttaattctagttcctttctggattcagatgcagaaacaatctcagctttcaaatcttccactgtactaagggacttatgtgcttcattaagtttactttcttgttcagctattgtctgtctagctctctgaatctgttcccttgaaaagctcaattcttcaacaaggtcttcaagctgtctctgtagagcacacttttcttctaaaattagtcctagttcttccttgagtttttccttttgagagttagtatcttgcaattttatattcagttcatttattgccacattcattaactttatctgatcttcattaactgtaatatttgaatatgaccttaaagcattctccatttctcccttatgccgtgttttcatttcctccatctgtgccatgtgttgtcttattaattcttgtttcatttgcactatctgctgcccatacatctcatccagctctgcccggagttgttctaactttctttgtgtttcttgttccattcgttgtactatatcagtttcgaactggctgtctttatgatttctcttctgaagttcttcgactgtccccattaactgttttatttcttcagaagactgtctttctttttgcttagaattagtcagctctaatttcatgttttttatttcttggttcttttgcacaatctgttcttgtaattctcctagtaatttatcagcagttgttaatttatcctttagctcaagagttttcttttcttcttctattatttttgtgtttaattcttcaatgattgtctccttttcctgtatttcttctttatttgagttttctacttttttatcttgttccatttcatatactttaattttctcttgcaagaaactaatttgcattgtgaagtcttctttctttttctgataatcttctaataagtggtcttgttcttcaagctgctgttgatgagtgaggatctgttgtttggcttgtagtaagtctgcagctgtgctactatgagtgctgtttctcagagtttcactagcctgtaattgctgaaattgaatctgtaatttttgactctgttctgtcaactctaaaaattctctcattgtctcatccttttctcttcttgcttgttgtaaattagcagtgagctgggttataatgccatctctttgtttaatggcagcttcaaattcttgtaactgctgcagtccttcagtcccataggtaaccctcatttcttccagctctctgtttagctcttcaatctcatgctgcttcccagccaactcactttccatcatctctagatgagtcggactgtcttgtgctccttgttcagaataagaatcatcaacaccaaattcttcttcccttaataaatttgtaggctttcctgttctcatcacaaaactgcaaccatttacctctgaactgcagtcatctgctgtggttgaaatttcactttccagttccacagagaagccctgctcatgactggttatttctccactatgtagagttctcattattgtagattcaggaatcacagttgattctactctctgagaactatttatgtacatttcattacactgtgattgatcaatattcaaatcatggtgtgctgacacatcatgtttactgcttgacgtttttctcttttttttctgcttcttggaaggactctgcccatccgactgagcttttctttgtcgaaactgggcaagcttggctttgccggcctccagcttcttctgtctctcctcgtcctccatggcctctgcaaggaaggcaggggaaaacaggggttgaggggtggttggggatagaaaggaaaggtcgatttggacggaggtgggacggcaagctccacggcctagagagccgattcggtccggcgctcccccgcccgaagtggaagcagtctccgcgctcactggcggatcgtcctcagccgcacgggaagcgccgtcaccgccgccgccgccgccatcttcgtctccacgta

SEQ ID NO: 14138 - RNA, 15775 nt, Homo sapiens
  source 1..15775: mol_type = other RNA
gctgggattacaggcatgagccaccgcacctggccttccctgcttcctctctagaatccaattagggatgtttgttactactcatattgattaaaacagttaacaaacttttttctttttaaaatgtgagatcagtgaactctggttttaagataatctgaaacaaggtccttgggagtaataaaattggtcacattctgtaaagcacattctgtttaggaatcaacttatctcaaattgtaactcggggcctaactatatgagatggctgaaaaaataccacatcgtctgttttcactaggtgatgccaaaatattttgctttatgtatattacagttctttttaaaacactggaagactcatgttaaactctaattgtgaaggcagaatctctgctaatttttcagattaaaattctctttgaaaaaatacagtctgtattcatgaattgtaaaatatgtgcttcagtgagcagagttagggaatccaggaacttgggtggggaaaaattacatctttatttgcactaataatttctaactgcaatttagtatttatttcaattatgaatttgggcagcattttattagcagtatccatgattttgtcaatagaaatctcagatattttcatattacagatgttacagatttcttgaagtatctagttacgaccccgagataaggctagtctaatgtttagtgaatagttttagacttcttaacagatttcatttttaatcacagactaattaattattgagatgcataaacaagtgtgattgcagaggcctactatcataaggaggcgtggtggtcaaacaatggcactgaactcagcttgatcagatcatttgtccatctgtttttttctccactgtctcttagagcagaatagccttgaatggcaagccatgctagctgaaaaaggtttttacccacaacctgccccttcaactaactgctttagagtacgtttgctatttttagaattcctcttattggaacccagcttctaatgtggaaaatttaagtatagttggctccttttatttgtgggttctgtatcctctgattcaaccaactgcaggttcaaaatactaaaaataaaaccccacaataaaaaaatacagtattagcaactatttacataatgttcacattgtattaggtatcaaataatctggagatgatttgaagtacacaggaggatgtatgtagactatctgcaaatagcacattgttttataagagacttaagcattcgcggactgtaatatccaagggggatcctggaactaatcccccacacatgccgagggatgactgaaattagaaatgttcaagcatgtacaactttctaccatgcctgtttgtgttggtataaatcatggaacatcaaataataagacaaaatcctccaggtgtaagcatcaaatactagtcctcttgctgttttagtgagttgccatgttattgaggaggactccagatgagaaataacattgcgatctgtattatctctgtgagagcctcccagtctgaatttggcttggacaacagggatactgtttaattcggctgcaatgtgattaagatcttttgagttaatgatttcttcatctttttagtgggccatggatttgtgagaacacatctttggaaacaagtaacactaactgtaatatagtaaatactgattaatcatgaaataccaatatagcttttaaaaaacactatgtagatgtaaagttgatacaaagacacatggaaaactttcaacagtattaactctaagattaggacaactttctctgaatctctcactcctacatatttgacataagtaatgagatgctatgtaccaagaactatggctcagttaaaaatgaagaaggttcaaatacagtgtggtgaaaatggtgaagtcatttttatttcagtacttgacaaaataccccataaaattcaaaacttctaccattatacaaaaataggtctctacaagtgatattatctgtcttcatcaccagtagaatatattaggcaaaacatgtaacttcagtagccttataagaaaagtgcaggacacctcgagctacacattcagcagtattgtaatgcgtaaaagtttaatcttttcacccatttgataaatacacaaggtttataatttaatgttttaaattagcattccacaaatatacaggtaattcaataattattgtgcatgaatacatacacaatgcttatatatacaaattccagtttgttttcatgtgctggcaagggatttgtatacaatcataagctgtgttcatattggtcccattgaatattcacaatacaaaagcacaaaagaaccattgatttacaaaaggaaatctatttaaaatcacttcaattaatgatgtttcaaaggattatcttctcatgccagcatgaaattgagtagttgaacctatgagagaaaaacaggaaattcaactgatttcaaattacattgctacctgtatcagacccaccagagttcacacaaaggaaattattattattctccatttttttaaagccctttttttccttaaaatgtcctcttcatacttaaactgagtctctccccactacccccaaggtggagtgttactctgttgcccaggctggaattcagtggtgtgatcttggctcactgcaacccccgcctcctgggttcaagtgattctcctgcctcagcctcctgagtagctgggactatccacacatgccaccatgtccagcaaatttttgtatttttagtggagacggggtttcaccatgttggccaggctagtctcgaactggttggtcttgaactcctgacctagtgatccgcctgcctcggccgcccaaagtgctgggattacaggcatgagccaccgcgcccagcccatatacttaagctgacttttaagagattttgaatatatatgtaaaaatcaccatgactggctctatggcaaggtaggtgagactaatatttagagtttttttaaagtgctctcaaagttggatgttctatacctcatacatttttgaaaaatcttttggtcttcaaaatctgggtcttgtgaaatttggatgctcaaaacaaaacaagcctaggcaaaccaacaaactcagctatgataataaaagtttcctattactacaagatgcttgggtgtaaacaaatgatttcttgaaggaagagataaactactcaatgattcaaagtctctgaatcaggagtgaactgaagtgagatagggaaaagaggttttccttccatgaacagggaatccacctttattttaaagtatgacttgttttttgtttttgaacaaagaaaaaataatccttacaaagtattttaaatgggatagtttttttcgatgatacataaaagcacaatatagtagcagggataatggttacattaagtgcttaaagtaagtgcttcctccttaactccacccgatttgcatgccttaccactttcttttttttttttttttctttgagacagggtctcgctctgctgcccaggctggagtgctgcggcacggccttaccactttctgccatgcgctacttaggaatacgttctccagttaggctctgtagactcagagtaccttgcacactggtgctcattgtgcattttgtgtcatcagtccgctgaatgaacatagtaggaaatcatttttgggaggagtgggatctggggtgataaatcatattttcacttaaattatttaaagtcagtttctctgctggttacaagagtttaagctttggctaacttaataattagctcatgcactaaactggaagctttgattatcctaatgagtgtgaaagaatttcaaagaaaggggagctgtgggtctcgcactgtggtgctgccaagatgtggttaaactcagagcacctgactgtatagttccaagtcgtctttgcagtgcctctagccgagtgatataatctgttagggctctgtcaggatcgtaattctgaagctgagaacatgctaaagaaccaggattgaaatcagctggagtgcctgggtacctattctgaaatggtaaaggggacctaatatagtccagatctgatcttgagcgatacgtagtatgtcttggttctccatataactccagcccaccagaagaatgataaaatgagtcagtcttttctgcaccttgattcagtccaaagccatctctgttaatattgatggaaacagaacctgtgactcgatgccaccgtcgaaccaaaaatttcattctggaaattgcaatggatactctgacggccgaccgaaacctggtgaagccctttgggcgattggtgatcacctctagatccgtgaaagctggctgcccccccatccgggcaagcagggccaaggtggcatcttcacattcctggaacccacccagtaacagcagcaggtatttcttctggtaaatgagagcctttcgaaaactttctgccctcaagtatttaccataaattctctttaaagtgacatgttcagaatcagggctcagagtttgaagtaaagagtcatttcttagttcagctttcagtttgtatacttcagcctctgcccttttcaaagatttctggagagtcaatttttctctgttccatacttctttttcagaggcaatgatggcttcaatgttggcaccaccattcaatgaaaacctggaagaattatctctaccagctcctgtctgtcgataccacctgatctgctcttccagcttcataaccatgttccttaagtcattcttctcttcagtcagttgactgatatgccctgtcagctcagcattttgtctcagtagtctttcagtcaatgagccacaagaagtacttggggacaccaagctgggctcttcaccttgctggccagttaatttctgtagttgtaaaataatttcatcaatattttcctgaacccaaatgaaatcttcatcatctgctgtttcaaactgtagtctctcagaggctttctggggtagaacctgtagttttgaagctacacattgaagcttttgtctgatcatttctaattcatgattacagccggttcctcctccattcatttcaatcaatttagcgtagtttgattcttttgtttctccttctattttctgttgaagaacccaatttctagttctatcactggttaagctccacgtggttggctcattaaggttctgatacagaattcttctactttctcgtttttcttctcgttctagttcttgcttctggaattcctgcatgattccttgtagtcgctgtccttcaaggtctaacttataaacttgttgtcttttctcttccagctggcgctgaagatcttccactttggactggagctcatgcatttttttctgtccctcagtgttggcctcctgttctgtctgcagtgttttcctgtgaacctgcctatctttttccatttgctgtcgtgtttgcaaagaatccagtttatatttttcagtctcatttaacaattctactatgcgactgtgtttttcctctagctgtttctgcagctctttcagtaggtcctctgagggcaagggtggccgagactgtccagtaccatcactgctctgcagctgtgcgtgcaattcccgctccctatctagggtactactcatttcccgaattcgaactttctcagattcaagaagtacctgaagctctaagtttcgaccttgttcttctgacaactgggcatcatatagcattctctgtgattctattttttgctgggattcgttcagtagttgtttctgttgttccaaaagtagatttagctgaagattcctttgtttctgactctcaagtgaaaacttcagatcctcaagttcttctttatcccgttcttcactgcgtcccaacttggctttctctttctccaaagcccactggagctctcttgattttttctgttcacttgctaatgtgtcattaagcaaatgtacttcatctgtcttatctttaacttccaacctgaaagcctccaattcttttaggtgtttatgctgtgccttgagtgttgtttctagttccaatttagtttgtgcaagctcactcttcagttcagcaaccaccattttctcagaactcagctgctcctgcagttccgttgctctgtctttcatactgctgagctccacttgcatctccagcatttgagactgcttctgctgtatattatattccaagagttcttggcttggtttctcactctcttgttctcttttcagagtaattttcctaccattcatttgtgcatgcagtgcctgaatttcagataacaaactccttctatctgctttctggaggcattccatagctgcttgatattcaacaccctgttcttgtattctctgttccaaacagtttagtaaaccaactgcatctgtagtacctagagctgtcagctccgtccgaaatgctgctagtaaaacactacgctcttctaagaaaacttgttgaagggcaagcagtagttcacctcgccagtctgagaagctctcatgagattgagaactatcataaacctcggcttctctttgcagttgcatctttgtaattaaatcctttagagatgagattgtattgatgtaagcttttctctcttctagccaaggttctgaaacctgctgaatagaatggtcctctccatcactatagggagactcagtgagagaaagcacctgcatgccttcattatggacagctctcagtaatccctttattttctttggaaaggaatctgttgcactttcactttcttctcctcggccttctgatgctatgtcaaatccctgactgtgtgtaagataaattccctgaccccagtctgatccagaatcactggagcatatttctctagtctggtaagcatcagaatgtgctagctcaggaattgaggatccctctttacttctcagacactgtatcactgccttcaaggtaccacattcctctttcagtaactgaacggcaacatagtgttccctctttaaggtttcagtttctgaaatatgtctggattccatgtccaaaatttcagcagcatgtagttcttgcatcttctcaattttttcagtaaactgactgattatttcagtaacttcttctgaggaacattcactctgtaaattaatttgtattcctgcatttttaacaagaatttgtggagtctgattgctgctactgatcttcagagtcccatctgtctgggatgcaatgctcttactcagttttataggaagtggctcaaacatgcaggcctttttgctttcttgtacctcagtctcatcttctttttctaaaatggacaatttctcttttgcctctgcgaggtgatccctaacttggcttaagtctttctgaagagatgtcatatttgtttcttttaccaaaagctcttcttgaagtttttcagccttttctttataactggcaagttctgctttggtagccactgattcagctctaagagcctcgagttcattaaaaaatccactttcttcattgctatgaaatagctcagtagttgtcttgagaacttcaacatcttgagggcttcttttcttttctttctctctctgttttttctcattgccctccaatagcttctgtagttctagcagcttcttttctttttctaaaacatttttttctgcaatttctacttgttctttttctaaaatcaaactagtatgcatttcaacaacctggctttctaattctgatattctcaaggttaatgctgatatatctgaccccaactcatcttctcttagttgatttaaattctgaatatttgttctttcaggttctgatgaaattgtttgattatcttgacagaattttgcatattcctgaactgcctcaagttggatttgactgacaagagcagcagccactttttcttcaactattttctgtaggtttacaatcttcttttgaagcatttctgtttcaaactggccttgttcttgcatgtcttttatttgtttataacactgggtaagttctaagtcctttgcactaacagtgctctcaagttgtagcaaccttgtttccaaattaattatggaacctttgccattttcttcaaaagatttgaagtatgtctgattttctagggatttaagagcatcctctgtaaggactacttctagttcaggtttgtctttgctcagatgatctatagccacgttaacactattctctggtatgctttgaatcttttccacactttcacgttctctctttaagctgaataattcctgtgttagctgattcattttaaaattggtttctttaagtacatttttcatgaaggtcatttcttcattagcggtttctacttgctgttccaaggccagcttttcagctataaccacatccaattgatgttttaaactgtctgcttcttctgagagggaatgagcattcattgatgtcttctgtccaatatttgccaattcctgttgaagtttttcaatcacttcattgagctgctctatttcttcttctctatttctcttcacacattcttgatcactcatcaaacattctatttgggtttcaagatcccttatcagttcatttttttcttcaataaccttgttatctgttgtaattttaagttgctgctggagtttcgtaacttgttcatttaattggtcaatttctacctctttttcctgtattatttgagcaaatttcccaaatagcacatgttggtcttgagtagacatggcatcagattcctttatggcaagtcccagtttctccatgtcatccttaaataatttgttttcctgttcaagttcttgtaggcgggtagtagattcctttttctgtatttctaattgcatatgtaattgttgaacttcttcattcttattttccagttcttctctaaactgttctaattgctcttctaagtttgtaatctctttttcctttctgtctatggcatctcgttcagcctgcaattgtacttctagggacaattctggtttagcttctacagctccaaagtgttttcggtcctctaccttttgaaaagtatctgcactcacaagaagcgcctgctccagttctcttactctgaactccagtttctctatttcttcattcctttcttgtatatccctttgaagctgctctttagagagcaaaagctcactgcatttgtctgttttttctttcagatgatttgctaactgttcaacctctctagtttgatgttcactgataggctggaatcgaggaacaaccttaagttgctgttctagtttctgtatttcctgttggaatacatctctctcatgttctctgtcaatggcttgctcatctaaaaattttctcattttttctaactgcttttccaatgcttggttttgctgtcttaaatccattagttcagtatttttttcttgttccagctctataaacctactgacttgttcttccacatctatttctagagctttcacttgtttttgaaggtcatcacgtactttttcagcttgacattgtacttctagtttttccttcattaatttttctgtctcctgtagtaattgttgttcaactgggcctgcctctgctttcatagcttccttttgtctggacagtaattctctttcttcttggatctgctgttgctctgcctccaattcttgcaacctgttacttgcacataacaactcctgctcaagacgatctattatatcagttttttcctgaatttgcctttcaaaaagagttttttcatctgcatagccatcaatgacgccctcagccttactgagctccacagctagctgttctctggccctggactcctcatgaaggcgctctcgaagttcctcttggcacttaagggactctgttgcttcttgtttctgtctaaatgactcacgcatcaactctgtctgtgtcactttcgcatgttcaagctgactgctagtttcacttatggcttctaggagtttttcaactgctgcttgtagtcgagagctaatgttcagcataagttcttcattttcagggtctatttcagttccagcaaaaccactcctcacaagtcgttgtgacagctctgttccttcctcagttacttttgaccacatgttaatgtcatttcttggcatatcacttccagaataagagggaatggattcatctgtaactcttgtatgttcctcatggacacatgactttacagatgcctctgcttctgacctccaaattaggctggcagatgactggcttttactagatctatctagaatcccaaggacatggcgaccaattgtttcttcaacagctgctgttgtctttacaacttctaagaggatcttcaaaagtctattattagctttctggagtgcatacctttcattagacaaaatctcaggaggcacatcttcaggttttctgtctaattccttttctttaaatgtttgttcttcaacttctccttggttttcatttccattctgtgtttgcgtactgctgttgcgcagctcacaacacagcttctctcttccagctaaagacagctgctttagtgcttccagctcctctaaaagcaccctctctctctctgaaaccaggttttcattatctatggaggatctctgggctaattgtctattaagtctcttaatctcttcttgtagctgttcctggtcttctcgctgtctctccatttgccgcatatgtgcttgccttaacaattccgttgcctgttgatgttcttggtattgtcgtacaagttcctgtctcatatcttccaactgttcttcattcaacattagttgtctagaagcatccatgcttgacactgaaatctcatcatgaatagactgtctaactataaatgttttatctttggagaacatttcttctgaaatagtcagcacacagtcctttgattctggtatatcatggggatcactatttgataataaaatttcctttccatgttctcctaactctttactaagtggtttaaattcttctttaaatttcacatccactgtctcaaaagtctgaaaaccaatttgatcctgtgataatttcatttcattaaaataatgttgttcttgctgacacacagcatgtgcttgctttgatgatgcagtattttcttttcccccagatattctagacagttcagtttgttgagcaaatgctatactcattgacacaataacctctattgtaccatcaatattctttttcacacaacttccagggtacattgttctctgtgcatcagattctgtaattaccaccgaatcaacaggtaagcttggcggaaccgtggactcactaacagcttgaagcctcttctgtaaacagtggatctctgcctcatagttttgttcagtttctttcaactgttgctgcaaagaggatatgaggctttctaattcttgaacttgttcttcaagtttagttttttcaagatcttgcagagaagataacttgcttttatgattgacatcaatgtcttccaaattggtcatctgagaatggattgataaaaactctgtttcctcttttggaaggttttcttctccaaattcaagtttcataccatctgtctgctgtccccagatcttgcttagtcgtgtttgaagtaccaagagtttgttgtattcttctgttactttgttgagaagagtgtgcatattttcttgaaagtcttgaacttcatatctataatcttgtaattctggatcttcattttcagaaatgtaatcaccagaattctctttgtcttctgcatttacttcacattttaaagcaggagtataatattcaccaaggacactgcataaagtctgtaaaaaataagaacattcttcagacactgccttttgaagttttccaatgagcagatgtaaaggctttccttcatcacctgtttcttgtgttttcatagtctgtagttctaactggtgtattttctgaagttccttgatcttttcctcttgagcaaaaataagctcttctttaagactgcaaagagctttatctttttcattttccatatattcacgaacctgatccacatgagttgaataaaccagagagaggcaaatgcgttgggcttccatctgtagccttaaatcattctgttctgatttaagtacattgagttctttctgaagtttatcattttcacttggttgagttgctctaagtgatgattcctttgttacagatggtaagtgatccaaaatcaactgttcttgcttactttcttctccaacagtcatattttcaaaagaaactttatcttccaccattatttttgattcttcaccaaaacttttatttactttagaaactgatccttcagcacccctgcttgtcatggtcacaactccatctaataaagagcttacttgagtatcacatgactgtacattttctgccctgttgtggttaataatgatttctagctctctacatctcaatgaaacttgttctttctcttgctttaaagatttaacttcttcatttagaaaactaatctcaccatgtttctgtttcaattgttcagaaagatcagacagtctctgtgacagctctaatttctctcgcttggttacctcaagtttttccatgagttctgttgtatccttttcaacaacctcacccatttccaatgtttctgctacaaaagttttgtcttcatcaaagacagaacttttcattttcactgtagttggatttattctttgcaaatgaagctcttcattaagtgctttaagtttacttttatactctaattcctgtttatttttactgtcttctaaatcatcttttactttgagaaggcaagcatactcctcttgtaactcttgatagttaacttcaaagtttttttcagcaaatgaaaaagtgttcctttgcttttcaatctcttcatttagctgaatacattgttgtttgaggtcctcattttcctctataagtatttctatttctttttcccacacagagtctttggatttggacttaatggagtctaagaaaatcaatctttcttcttggctaacaggagtatgtattttcaacatgtcttcaagggttttcttttcatctttaagaatgctattctctgcttcaagttgtgcaaatttttcttgaagatcattctctttttccttcatctgtttttctaacaattctgttttaagttgtaattcttgaacttcttgttcaagtgtacccttttctttttcttcttgtctgagtatttcaatttctttttgaagttcattgatttgaagagtcatttcttctgactttgaatttacaagagactgctgtaaatcttttagctttgaaatttccaaaattaattgattctgcttagttatcaaattgtccttttcaaactgcatggtttctatcttttgactcatttcattctgtaaaccatctatctgctgtttatagtgaatgcctaaattatctttaagtttttcaatatttattcgatgttcaatttctaaatcttccttcagtttggaaagctcttcttcgtgactaaatagaagctgtgttctcagcctctctaattcagcttcttgtgattcagccattctgtctaacacagcattcttttctttttctaacatttcaagttttatcttgtaatttgtaacttctgcttcatgttttaattctagttcctttctggattcagatgcagaaacaatctcagctttcaaatcttccactgtactaagggacttatgtgcttcattaagtttactttcttgttcagctattgtctgtctagctctctgaatctgttcccttgaaaagctcaattcttcaacaaggtcttcaagctgtctctgtagagcacacttttcttctaaaattagtcctagttcttccttgagtttttccttttgagagttagtatcttgcaattttatattcagttcatttattgccacattcattaactttatctgatcttcattaactgtaatatttgaatatgaccttaaagcattctccatttctcccttatgccgtgttttcatttcctccatctgtgccatgtgttgtcttattaattcttgtttcatttgcactatctgctgcccatacatctcatccagctctgcccggagttgttctaactttctttgtgtttcttgttccattcgttgtactatatcagtttcgaactggctgtctttatgatttctcttctgaagttcttcgactgtccccattaactgttttatttcttcagaagactgtctttctttttgcttagaattagtcagctctaatttcatgttttttatttcttggttcttttgcacaatctgttcttgtaattctcctagtaatttatcagcagttgttaatttatcctttagctcaagagttttcttttcttcttctattatttttgtgtttaattcttcaatgattgtctccttttcctgtatttcttctttatttgagttttctacttttttatcttgttccatttcatatactttaattttctcttgcaagaaactaatttgcattgtgaagtcttctttctttttctgataatcttctaataagtggtcttgttcttcaagctgctgttgatgagtgaggatctgttgtttggcttgtagtaagtctgcagctgtgctactatgagtgctgtttctcagagtttcactagcctgtaattgctgaaattgaatctgtaatttttgactctgttctgtcaactctaaaaattctctcattgtctcatccttttctcttcttgcttgttgtaaattagcagtgagctgggttataatgccatctctttgtttaatggcagcttcaaattcttgtaactgctgcagtccttcagtcccataggtaaccctcatttcttccagctctctgtttagctcttcaatctcatgctgcttcccagccaactcactttccatcatctctagatgagtcggactgtcttgtgctccttgttcagaataagaatcatcaacaccaaattcttcttcccttaataaatttgtaggctttcctgttctcatcacaaaactgcaaccatttacctctgaactgcagtcatctgctgtggttgaaatttcactttccagttccacagagaagccctgctcatgactggttatttctccactatgtagagttctcattattgtagattcaggaatcacagttgattctactctctgagaactatttatgtacatttcattacactgtgattgatcaatattcaaatcatggtgtgctgacacatcatgtttactgcttgacgtttttctcttttttttctgcttcttggaaggactctgcccatccgactgagcttttctttgtcgaaactgggcaagcttggctttgccggcctccagcttcttctgtctctcctcgtcctccatggcctctgcaaggaaggcaggggaaaacaggggttgaggggtggttggggatagaaaggaaaggtcgatttggacggaggtgggacggcaagctccacggcctagagagccgattcggtccggcgctcccccgcccgaagtggaagcagtctccgcgctcactggcggatcgtcctcagccgcacgggaagcgccgtcaccgccgccgccgccgccatcttcgtctccacgta

SEQ ID NO: 14139 - RNA, 15868 nt, Homo sapiens
  source 1..15868: mol_type = other RNA
gctgggattacaggcatgagccaccgcacctggccttccctgcttcctctctagaatccaattagggatgtttgttactactcatattgattaaaacagttaacaaacttttttctttttaaaatgtgagatcagtgaactctggttttaagataatctgaaacaaggtccttgggagtaataaaattggtcacattctgtaaagcacattctgtttaggaatcaacttatctcaaattgtaactcggggcctaactatatgagatggctgaaaaaataccacatcgtctgttttcactaggtgatgccaaaatattttgctttatgtatattacagttctttttaaaacactggaagactcatgttaaactctaattgtgaaggcagaatctctgctaatttttcagattaaaattctctttgaaaaaatacagtctgtattcatgaattgtaaaatatgtgcttcagtgagcagagttagggaatccaggaacttgggtggggaaaaattacatctttatttgcactaataatttctaactgcaatttagtatttatttcaattatgaatttgggcagcattttattagcagtatccatgattttgtcaatagaaatctcagatattttcatattacagatgttacagatttcttgaagtatctagttacgaccccgagataaggctagtctaatgtttagtgaatagttttagacttcttaacagatttcatttttaatcacagactaattaattattgagatgcataaacaagtgtgattgcagaggcctactatcataaggaggcgtggtggtcaaacaatggcactgaactcagcttgatcagatcatttgtccatctgtttttttctccactgtctcttagagcagaatagccttgaatggcaagccatgctagctgaaaaaggtttttacccacaacctgccccttcaactaactgctttagagtacgtttgctatttttagaattcctcttattggaacccagcttctaatgtggaaaatttaagtatagttggctccttttatttgtgggttctgtatcctctgattcaaccaactgcaggttcaaaatactaaaaataaaaccccacaataaaaaaatacagtattagcaactatttacataatgttcacattgtattaggtatcaaataatctggagatgatttgaagtacacaggaggatgtatgtagactatctgcaaatagcacattgttttataagagacttaagcattcgcggactgtaatatccaagggggatcctggaactaatcccccacacatgccgagggatgactgaaattagaaatgttcaagcatgtacaactttctaccatgcctgtttgtgttggtataaatcatggaacatcaaataataagacaaaatcctccaggtgtaagcatcaaatactagtcctcttgctgttttagtgagttgccatgttattgaggaggactccagatgagaaataacattgcgatctgtattatctctgtgagagcctcccagtctgaatttggcttggacaacagggatactgtttaattcggctgcaatgtgattaagatcttttgagttaatgatttcttcatctttttagtgggccatggatttgtgagaacacatctttggaaacaagtaacactaactgtaatatagtaaatactgattaatcatgaaataccaatatagcttttaaaaaacactatgtagatgtaaagttgatacaaagacacatggaaaactttcaacagtattaactctaagattaggacaactttctctgaatctctcactcctacatatttgacataagtaatgagatgctatgtaccaagaactatggctcagttaaaaatgaagaaggttcaaatacagtgtggtgaaaatggtgaagtcatttttatttcagtacttgacaaaataccccataaaattcaaaacttctaccattatacaaaaataggtctctacaagtgatattatctgtcttcatcaccagtagaatatattaggcaaaacatgtaacttcagtagccttataagaaaagtgcaggacacctcgagctacacattcagcagtattgtaatgcgtaaaagtttaatcttttcacccatttgataaatacacaaggtttataatttaatgttttaaattagcattccacaaatatacaggtaattcaataattattgtgcatgaatacatacacaatgcttatatatacaaattccagtttgttttcatgtgctggcaagggatttgtatacaatcataagctgtgttcatattggtcccattgaatattcacaatacaaaagcacaaaagaaccattgatttacaaaaggaaatctatttaaaatcacttcaattaatgatgtttcaaaggattatcttctcatgccagcatgaaattgagtagttgaacctatgagagaaaaacaggaaattcaactgatttcaaattacattgctacctgtatcagacccaccagagttcacacaaaggaaattattattattctccatttttttaaagccctttttttccttaaaatgtcctcttcatacttaaactgagtctctccccactacccccaaggtggagtgttactctgttgcccaggctggaattcagtggtgtgatcttggctcactgcaacccccgcctcctgggttcaagtgattctcctgcctcagcctcctgagtagctgggactatccacacatgccaccatgtccagcaaatttttgtatttttagtggagacggggtttcaccatgttggccaggctagtctcgaactggttggtcttgaactcctgacctagtgatccgcctgcctcggccgcccaaagtgctgggattacaggcatgagccaccgcgcccagcccatatacttaagctgacttttaagagattttgaatatatatgtaaaaatcaccatgactggctctatggcaaggtaggtgagactaatatttagagtttttttaaagtgctctcaaagttggatgttctatacctcatacatttttgaaaaatcttttggtcttcaaaatctgggtcttgtgaaatttggatgctcaaaacaaaacaagcctaggcaaaccaacaaactcagctatgataataaaagtttcctattactacaagatgcttgggtgtaaacaaatgatttcttgaaggaagagataaactactcaatgattcaaagtctctgaatcaggagtgaactgaagtgagatagggaaaagaggttttccttccatgaacagggaatccacctttattttaaagtatgacttgttttttgtttttgaacaaagaaaaaataatccttacaaagtattttaaatgggatagtttttttcgatgatacataaaagcacaatatagtagcagggataatggttacattaagtgcttaaagtaagtgcttcctccttaactccacccgatttgcatgccttaccactttcttttttttttttttttctttgagacagggtctcgctctgctgcccaggctggagtgctgcggcacggccttaccactttctgccatgcgctacttaggaatacgttctccagttaggctctgtagactcagagtaccttgcacactggtgctcattgtgcattttgtgtcatcagtccgctgaatgaacatagtaggaaatcatttttgggaggagtgggatctggggtgataaatcatattttcacttaaattatttaaagtcagtttctctgctggttacaagagtttaagctttggctaacttaataattagctcatgcactaaactggaagctttgattatcctaatgagtgtgaaagaatttcaaagaaaggggagctgtgggtctcgcactgtggtgctgccaagatgtggttaaactcagagcacctgactgtatagttccaagtcgtctttgcagtgcctctagccgagtgatataatctgttagggctctgtcaggatcgtaattctgaagctgagaacatgctaaagaaccaggattgaaatcagctggagtgcctgggtacctattctgaaatggtaaaggggacctaatatagtccagatctgatcttgagcgatacgtagtatgtcttggttctccatataactccagcccaccagaagaatgataaaatgagtcagtcttttctgcaccttgattcagtccaaagccatctctgttaatattgatggaaacagaacctgtgactcgatgccaccgtcgaaccaaaaatttcattctggaaattgcaatggatactctgacggccgaccgaaacctggtgaagccctttgggcgattggtgatcacctctagatccgtgaaagctggctgcccccccatccgggcaagcagggccaaggtggcatcttcacattcctggaacccacccagtaacagcagcaggtatttcttctggtaaatgagagcctttcgaaaactttctgccctcaagtatttaccataaattctctttaaagtgacatgttcagaatcagggctcagagtttgaagtaaagagtcatttcttagttcagctttcagtttgtatacttcagcctctgcccttttcaaagatttctggagagtcaatttttctctgttccatacttctttttcagaggcaatgatggcttcaatgttggcaccaccattcaatgaaaacctggaagaattatctctaccagctcctgtctgtcgataccacctgatctgctcttccagcttcataaccatgttccttaagtcattcttctcttcagtcagttgactgatatgccctgtcagctcagcattttgtctcagtagtctttcagtcaatgagccacaagaagtacttggggacaccaagctgggctcttcaccttgctggccagttaatttctgtagttgtaaaataatttcatcaatattttcctgaacccaaatgaaatcttcatcatctgctgtttcaaactgtagtctctcagaggctttctggggtagaacctgtagttttgaagctacacattgaagcttttgtctgatcatttctaattcatgattacagccggttcctcctccattcatttcaatcaatttagcgtagtttgattcttttgtttctccttctattttctgttgaagaacccaatttctagttctatcactggttaagctccacgtggttggctcattaaggttctgatacagaattcttctactttctcgtttttcttctcgttctagttcttgcttctggaattcctgcatgattccttgtagtcgctgtccttcaaggtctaacttataaacttgttgtcttttctcttccagctggcgctgaagatcttccactttggactggagctcatgcatttttttctgtccctcagtgttggcctcctgttctgtctgcagtgttttcctgtgaacctgcctatctttttccatttgctgtcgtgtttgcaaagaatccagtttatatttttcagtctcatttaacaattctactatgcgactgtgtttttcctctagctgtttctgcagctctttcagtaggtcctctgagggcaagggtggccgagactgtccagtaccatcactgctctgcagctgtgcgtgcaattcccgctccctatctagggtactactcatttcccgaattcgaactttctcagattcaagaagtacctgaagctctaagtttcgaccttgttcttctgacaactgggcatcatatagcattctctgtgattctattttttgctgggattcgttcagtagttgtttctgttgttccaaaagtagatttagctgaagattcctttgtttctgactctcaagtgaaaacttcagatcctcaagttcttctttatcccgttcttcactgcgtcccaacttggctttctctttctccaaagcccactggagctctcttgattttttctgttcacttgctaatgtgtcattaagcaaatgtacttcatctgtcttatctttaacttccaacctgaaagcctccaattcttttaggtgtttatgctgtgccttgagtgttgtttctagttccaatttagtttgtgcaagctcactcttcagttcagcaaccaccattttctcagaactcagctgctcctgcagttccgttgctctgtctttcatactgctgagctccacttgcatctccagcatttgagactgcttctgctgtatattatattccaagagttcttggcttggtttctcactctcttgttctcttttcagagtaattttcctaccattcatttgtgcatgcagtgcctgaatttcagataacaaactccttctatctgctttctggaggcattccatagctgcttgatattcaacaccctgttcttgtattctctgttccaaacagtttagtaaaccaactgcatctgtagtacctagagctgtcagctccgtccgaaatgctgctagtaaaacactacgctcttctaagaaaacttgttgaagggcaagcagtagttcacctcgccagtctgagaagctctcatgagattgagaactatcataaacctcggcttctctttgcagttgcatctttgtaattaaatcctttagagatgagattgtattgatgtaagcttttctctcttctagccaaggttctgaaacctgctgaatagaatggtcctctccatcactatagggagactcagtgagagaaagcacctgcatgccttcattatggacagctctcagtaatccctttattttctttggaaaggaatctgttgcactttcactttcttctcctcggccttctgatgctatgtcaaatccctgactgtgtgtaagataaattccctgaccccagtctgatccagaatcactggagcatatttctctagtctggtaagcatcagaatgtgctagctcaggaattgaggatccctctttacttctcagacactgtatcactgccttcaaggtaccacattcctctttcagtaactgaacggcaacatagtgttccctctttaaggtttcagtttctgaaatatgtctggattccatgtccaaaatttcagcagcatgtagttcttgcatcttctcaattttttcagtaaactgactgattatttcagtaacttcttctgaggaacattcactctgtaaattaatttgtattcctgcatttttaacaagaatttgtggagtctgattgctgctactgatcttcagagtcccatctgtctgggatgcaatgctcttactcagttttataggaagtggctcaaacatgcaggcctttttgctttcttgtacctcagtctcatcttctttttctaaaatggacaatttctcttttgcctctgcgaggtgatccctaacttggcttaagtctttctgaagagatgtcatatttgtttcttttaccaaaagctcttcttgaagtttttcagccttttctttataactggcaagttctgctttggtagccactgattcagctctaagagcctcgagttcattaaaaaatccactttcttcattgctatgaaatagctcagtagttgtcttgagaacttcaacatcttgagggcttcttttcttttctttctctctctgttttttctcattgccctccaatagcttctgtagttctagcagcttcttttctttttctaaaacatttttttctgcaatttctacttgttctttttctaaaatcaaactagtatgcatttcaacaacctggctttctaattctgatattctcaaggttaatgctgatatatctgaccccaactcatcttctcttagttgatttaaattctgaatatttgttctttcaggttctgatgaaattgtttgattatcttgacagaattttgcatattcctgaactgcctcaagttggatttgactgacaagagcagcagccactttttcttcaactattttctgtaggtttacaatcttcttttgaagcatttctgtttcaaactggccttgttcttgcatgtcttttatttgtttataacactgggtaagttctaagtcctttgcactaacagtgctctcaagttgtagcaaccttgtttccaaattaattatggaacctttgccattttcttcaaaagatttgaagtatgtctgattttctagggatttaagagcatcctctgtaaggactacttctagttcaggtttgtctttgctcagatgatctatagccacgttaacactattctctggtatgctttgaatcttttccacactttcacgttctctctttaagctgaataattcctgtgttagctgattcattttaaaattggtttctttaagtacatttttcatgaaggtcatttcttcattagcggtttctacttgctgttccaaggccagcttttcagctataaccacatccaattgatgttttaaactgtctgcttcttctgagagggaatgagcattcattgatgtcttctgtccaatatttgccaattcctgttgaagtttttcaatcacttcattgagctgctctatttcttcttctctatttctcttcacacattcttgatcactcatcaaacattctatttgggtttcaagatcccttatcagttcatttttttcttcaataaccttgttatctgttgtaattttaagttgctgctggagtttcgtaacttgttcatttaattggtcaatttctacctctttttcctgtattatttgagcaaatttcccaaatagcacatgttggtcttgagtagacatggcatcagattcctttatggcaagtcccagtttctccatgtcatccttaaataatttgttttcctgttcaagttcttgtaggcgggtagtagattcctttttctgtatttctaattgcatatgtaattgttgaacttcttcattcttattttccagttcttctctaaactgttctaattgctcttctaagtttgtaatctctttttcctttctgtctatggcatctcgttcagcctgcaattgtacttctagggacaattctggtttagcttctacagctccaaagtgttttcggtcctctaccttttgaaaagtatctgcactcacaagaagcgcctgctccagttctcttactctgaactccagtttctctatttcttcattcctttcttgtatatccctttgaagctgctctttagagagcaaaagctcactgcatttgtctgttttttctttcagatgatttgctaactgttcaacctctctagtttgatgttcactgataggctggaatcgaggaacaaccttaagttgctgttctagtttctgtatttcctgttggaatacatctctctcatgttctctgtcaatggcttgctcatctaaaaattttctcattttttctaactgcttttccaatgcttggttttgctgtcttaaatccattagttcagtatttttttcttgttccagctctataaacctactgacttgttcttccacatctatttctagagctttcacttgtttttgaaggtcatcacgtactttttcagcttgacattgtacttctagtttttccttcattaatttttctgtctcctgtagtaattgttgttcaactgggcctgcctctgctttcatagcttccttttgtctggacagtaattctctttcttcttggatctgctgttgctctgcctccaattcttgcaacctgttacttgcacataacaactcctgctcaagacgatctattatatcagttttttcctgaatttgcctttcaaaaagagttttttcatctgcatagccatcaatgacgccctcagccttactgagctccacagctagctgttctctggccctggactcctcatgaaggcgctctcgaagttcctcttggcacttaagggactctgttgcttcttgtttctgtctaaatgactcacgcatcaactctgtctgtgtcactttcgcatgttcaagctgactgctagtttcacttatggcttctaggagtttttcaactgctgcttgtagtcgagagctaatgttcagcataagttcttcattttcagggtctatttcagttccagcaaaaccactcctcacaagtcgttgtgacagctctgttccttcctcagttacttttgaccacatgttaatgtcatttcttggcatatcacttccagaataagagggaatggattcatctgtaactcttgtatgttcctcatggacacatgactttacagatgcctctgcttctgacctccaaattaggctggcagatgactggcttttactagatctatctagaatcccaaggacatggcgaccaattgtttcttcaacagctgctgttgtctttacaacttctaagaggatcttcaaaagtctattattagctttctggagtgcatacctttcattagacaaaatctcaggaggcacatcttcaggttttctgtctaattccttttctttaaatgtttgttcttcaacttctccttggttttcatttccattctgtgtttgcgtactgctgttgcgcagctcacaacacagcttctctcttccagctaaagacagctgctttagtgcttccagctcctctaaaagcaccctctctctctctgaaaccaggttttcattatctatggaggatctctgggctaattgtctattaagtctcttaatctcttcttgtagctgttcctggtcttctcgctgtctctccatttgccgcatatgtgcttgccttaacaattccgttgcctgttgatgttcttggtattgtcgtacaagttcctgtctcatatcttccaactgttcttcattcaacattagttgtctagaagcatccatgcttgacactgaaatctcatcatgaatagactgtctaactataaatgttttatctttggagaacatttcttctgaaatagtcagcacacagtcctttgattctggtatatcatggggatcactatttgataataaaatttcctttccatgttctcctaactctttactaagtggtttaaattcttctttaaatttcacatccactgtctcaaaagtctgaaaaccaatttgatcctgtgataatttcatttcattaaaataatgttgttcttgctgacacacagcatgtgcttgctttgatgatgcagtattttcttttcccccagatattctagacagttcagtttgttgagcaaatgctatactcattgacacaataaccttagctacttcttcttctaattgttcttggtattgtttttcaagcaacttaacgatatttgtttcctctttcactccaaattcaccagaaaactctattgtaccatcaatattctttttcacacaacttccagggtacattgttctctgtgcatcagattctgtaattaccaccgaatcaacaggtaagcttggcggaaccgtggactcactaacagcttgaagcctcttctgtaaacagtggatctctgcctcatagttttgttcagtttctttcaactgttgctgcaaagaggatatgaggctttctaattcttgaacttgttcttcaagtttagttttttcaagatcttgcagagaagataacttgcttttatgattgacatcaatgtcttccaaattggtcatctgagaatggattgataaaaactctgtttcctcttttggaaggttttcttctccaaattcaagtttcataccatctgtctgctgtccccagatcttgcttagtcgtgtttgaagtaccaagagtttgttgtattcttctgttactttgttgagaagagtgtgcatattttcttgaaagtcttgaacttcatatctataatcttgtaattctggatcttcattttcagaaatgtaatcaccagaattctctttgtcttctgcatttacttcacattttaaagcaggagtataatattcaccaaggacactgcataaagtctgtaaaaaataagaacattcttcagacactgccttttgaagttttccaatgagcagatgtaaaggctttccttcatcacctgtttcttgtgttttcatagtctgtagttctaactggtgtattttctgaagttccttgatcttttcctcttgagcaaaaataagctcttctttaagactgcaaagagctttatctttttcattttccatatattcacgaacctgatccacatgagttgaataaaccagagagaggcaaatgcgttgggcttccatctgtagccttaaatcattctgttctgatttaagtacattgagttctttctgaagtttatcattttcacttggttgagttgctctaagtgatgattcctttgttacagatggtaagtgatccaaaatcaactgttcttgcttactttcttctccaacagtcatattttcaaaagaaactttatcttccaccattatttttgattcttcaccaaaacttttatttactttagaaactgatccttcagcacccctgcttgtcatggtcacaactccatctaataaagagcttacttgagtatcacatgactgtacattttctgccctgttgtggttaataatgatttctagctctctacatctcaatgaaacttgttctttctcttgctttaaagatttaacttcttcatttagaaaactaatctcaccatgtttctgtttcaattgttcagaaagatcagacagtctctgtgacagctctaatttctctcgcttggttacctcaagtttttccatgagttctgttgtatccttttcaacaacctcacccatttccaatgtttctgctacaaaagttttgtcttcatcaaagacagaacttttcattttcactgtagttggatttattctttgcaaatgaagctcttcattaagtgctttaagtttacttttatactctaattcctgtttatttttactgtcttctaaatcatcttttactttgagaaggcaagcatactcctcttgtaactcttgatagttaacttcaaagtttttttcagcaaatgaaaaagtgttcctttgcttttcaatctcttcatttagctgaatacattgttgtttgaggtcctcattttcctctataagtatttctatttctttttcccacacagagtctttggatttggacttaatggagtctaagaaaatcaatctttcttcttggctaacaggagtatgtattttcaacatgtcttcaagggttttcttttcatctttaagaatgctattctctgcttcaagttgtgcaaatttttcttgaagatcattctctttttccttcatctgtttttctaacaattctgttttaagttgtaattcttgaacttcttgttcaagtgtacccttttctttttcttcttgtctgagtatttcaatttctttttgaagttcattgatttgaagagtcatttcttctgactttgaatttacaagagactgctgtaaatcttttagctttgaaatttccaaaattaattgattctgcttagttatcaaattgtccttttcaaactgcatggtttctatcttttgactcatttcattctgtaaaccatctatctgctgtttatagtgaatgcctaaattatctttaagtttttcaatatttattcgatgttcaatttctaaatcttccttcagtttggaaagctcttcttcgtgactaaatagaagctgtgttctcagcctctctaattcagcttcttgtgattcagccattctgtctaacacagcattcttttctttttctaacatttcaagttttatcttgtaatttgtaacttctgcttcatgttttaattctagttcctttctggattcagatgcagaaacaatctcagctttcaaatcttccactgtactaagggacttatgtgcttcattaagtttactttcttgttcagctattgtctgtctagctctctgaatctgttcccttgaaaagctcaattcttcaacaaggtcttcaagctgtctctgtagagcacacttttcttctaaaattagtcctagttcttccttgagtttttccttttgagagttagtatcttgcaattttatattcagttcatttattgccacattcattaactttatctgatcttcattaactgtaatatttgaatatgaccttaaagcattctccatttctcccttatgccgtgttttcatttcctccatctgtgccatgtgttgtcttattaattcttgtttcatttgcactatctgctgcccatacatctcatccagctctgcccggagttgttctaactttctttgtgtttcttgttccattcgttgtactatatcagtttcgaactggctgtctttatgatttctcttctgaagttcttcgactgtccccattaactgttttatttcttcagaagactgtctttctttttgcttagaattagtcagctctaatttcatgttttttatttcttggttcttttgcacaatctgttcttgtaattctcctagtaatttatcagcagttgttaatttatcctttagctcaagagttttcttttcttcttctattatttttgtgtttaattcttcaatgattgtctccttttcctgtatttcttctttatttgagttttctacttttttatcttgttccatttcatatactttaattttctcttgcaagaaactaatttgcattgtgaagtcttctttctttttctgataatcttctaataagtggtcttgttcttcaagctgctgttgatgagtgaggatctgttgtttggcttgtagtaagtctgcagctgtgctactatgagtgctgtttctcagagtttcactagcctgtaattgctgaaattgaatctgtaatttttgactctgttctgtcaactctaaaaattctctcattgtctcatccttttctcttcttgcttgttgtaaattagcagtgagctgggttataatgccatctctttgtttaatggcagcttcaaattcttgtaactgctgcagtccttcagtcccataggtaaccctcatttcttccagctctctgtttagctcttcaatctcatgctgcttcccagccaactcactttccatcatctctagatgagtcggactgtcttgtgctccttgttcagaataagaatcatcaacaccaaattcttcttcccttaataaatttgtaggctttcctgttctcatcacaaaactgcaaccatttacctctgaactgcagtcatctgctgtggttgaaatttcactttccagttccacagagaagccctgctcatgactggttatttctccactatgtagagttctcattattgtagattcaggaatcacagttgattctactctctgagaactatttatgtacatttcattacactgtgattgatcaatattcaaatcatggtgtgctgacacatcatgtttactgcttgacgtttttctcttttttttctgcttcttggaaggactctgcccatccgactgagcttttctttgtcgaaactgggcaagcttggctttgccggcctccagcttcttctgtctctcctcgtcctccatggcctctgcaaggaaggcaggggaaaacaggggttgaggggtggttggggatagaaaggaaaggtcgatttggacggaggtgggacggcaagctccacggcctagagagccgattcggtccggcgctcccccgcccgaagtggaagcagtctccgcgctcactggcggatcgtcctcagccgcacgggaagcgccgtcaccgccgccgccgccgccatcttcgtctccacgta

SEQ ID NO: 14140 - RNA, 10835 nt, Homo sapiens
  source 1..10835: mol_type = other RNA
gctgggattacaggcatgagccaccgcacctggccttccctgcttcctctctagaatccaattagggatgtttgttactactcatattgattaaaacagttaacaaacttttttctttttaaaatgtgagatcagtgaactctggttttaagataatctgaaacaaggtccttgggagtaataaaattggtcacattctgtaaagcacattctgtttaggaatcaacttatctcaaattgtaactcggggcctaactatatgagatggctgaaaaaataccacatcgtctgttttcactaggtgatgccaaaatattttgctttatgtatattacagttctttttaaaacactggaagactcatgttaaactctaattgtgaaggcagaatctctgctaatttttcagattaaaattctctttgaaaaaatacagtctgtattcatgaattgtaaaatatgtgcttcagtgagcagagttagggaatccaggaacttgggtggggaaaaattacatctttatttgcactaataatttctaactgcaatttagtatttatttcaattatgaatttgggcagcattttattagcagtatccatgattttgtcaatagaaatctcagatattttcatattacagatgttacagatttcttgaagtatctagttacgaccccgagataaggctagtctaatgtttagtgaatagttttagacttcttaacagatttcatttttaatcacagactaattaattattgagatgcataaacaagtgtgattgcagaggcctactatcataaggaggcgtggtggtcaaacaatggcactgaactcagcttgatcagatcatttgtccatctgtttttttctccactgtctcttagagcagaatagccttgaatggcaagccatgctagctgaaaaaggtttttacccacaacctgccccttcaactaactgctttagagtacgtttgctatttttagaattcctcttattggaacccagcttctaatgtggaaaatttaagtatagttggctccttttatttgtgggttctgtatcctctgattcaaccaactgcaggttcaaaatactaaaaataaaaccccacaataaaaaaatacagtattagcaactatttacataatgttcacattgtattaggtatcaaataatctggagatgatttgaagtacacaggaggatgtatgtagactatctgcaaatagcacattgttttataagagacttaagcattcgcggactgtaatatccaagggggatcctggaactaatcccccacacatgccgagggatgactgaaattagaaatgttcaagcatgtacaactttctaccatgcctgtttgtgttggtataaatcatggaacatcaaataataagacaaaatcctccaggtgtaagcatcaaatactagtcctcttgctgttttagtgagttgccatgttattgaggaggactccagatgagaaataacattgcgatctgtattatctctgtgagagcctcccagtctgaatttggcttggacaacagggatactgtttaattcggctgcaatgtgattaagatcttttgagttaatgatttcttcatctttttagtgggccatggatttgtgagaacacatctttggaaacaagtaacactaactgtaatatagtaaatactgattaatcatgaaataccaatatagcttttaaaaaacactatgtagatgtaaagttgatacaaagacacatggaaaactttcaacagtattaactctaagattaggacaactttctctgaatctctcactcctacatatttgacataagtaatgagatgctatgtaccaagaactatggctcagttaaaaatgaagaaggttcaaatacagtgtggtgaaaatggtgaagtcatttttatttcagtacttgacaaaataccccataaaattcaaaacttctaccattatacaaaaataggtctctacaagtgatattatctgtcttcatcaccagtagaatatattaggcaaaacatgtaacttcagtagccttataagaaaagtgcaggacacctcgagctacacattcagcagtattgtaatgcgtaaaagtttaatcttttcacccatttgataaatacacaaggtttataatttaatgttttaaattagcattccacaaatatacaggtaattcaataattattgtgcatgaatacatacacaatgcttatatatacaaattccagtttgttttcatgtgctggcaagggatttgtatacaatcataagctgtgttcatattggtcccattgaatattcacaatacaaaagcacaaaagaaccattgatttacaaaaggaaatctatttaaaatcacttcaattaatgatgtttcaaaggattatcttctcatgccagcatgaaattgagtagttgaacctatgagagaaaaacaggaaattcaactgatttcaaattacattgctacctgtatcagacccaccagagttcacacaaaggaaattattattattctccatttttttaaagccctttttttccttaaaatgtcctcttcatacttaaactgagtctctccccactacccccaaggtggagtgttactctgttgcccaggctggaattcagtggtgtgatcttggctcactgcaacccccgcctcctgggttcaagtgattctcctgcctcagcctcctgagtagctgggactatccacacatgccaccatgtccagcaaatttttgtatttttagtggagacggggtttcaccatgttggccaggctagtctcgaactggttggtcttgaactcctgacctagtgatccgcctgcctcggccgcccaaagtgctgggattacaggcatgagccaccgcgcccagcccatatacttaagctgacttttaagagattttgaatatatatgtaaaaatcaccatgactggctctatggcaaggtaggtgagactaatatttagagtttttttaaagtgctctcaaagttggatgttctatacctcatacatttttgaaaaatcttttggtcttcaaaatctgggtcttgtgaaatttggatgctcaaaacaaaacaagcctaggcaaaccaacaaactcagctatgataataaaagtttcctattactacaagatgcttgggtgtaaacaaatgatttcttgaaggaagagataaactactcaatgattcaaagtctctgaatcaggagtgaactgaagtgagatagggaaaagaggttttccttccatgaacagggaatccacctttattttaaagtatgacttgttttttgtttttgaacaaagaaaaaataatccttacaaagtattttaaatgggatagtttttttcgatgatacataaaagcacaatatagtagcagggataatggttacattaagtgcttaaagtaagtgcttcctccttaactccacccgatttgcatgccttaccactttcttttttttttttttttctttgagacagggtctcgctctgctgcccaggctggagtgctgcggcacggccttaccactttctgccatgcgctacttaggaatacgttctccagttaggctctgtagactcagagtaccttgcacactggtgctcattgtgcattttgtgtcatcagtccgctgaatgaacatagtaggaaatcatttttgggaggagtgggatctggggtgataaatcatattttcacttaaattatttaaagtcagtttctctgctggttacaagagtttaagctttggctaacttaataattagctcatgcactaaactggaagctttgattatcctaatgagtgtgaaagaatttcaaagaaaggggagctgtgggtctcgcactgtggtgctgccaagatgtggttaaactcagagcacctgactgtatagttccaagtcgtctttgcagtgcctctagccgagtgatataatctgttagggctctgtcaggatcgtaattctgaagctgagaacatgctaaagaaccaggattgaaatcagctggagtgcctgggtacctattctgaaatggtaaaggggacctaatatagtccagatctgatcttgagcgatacgtagtatgtcttggttctccatataactccagcccaccagaagaatgataaaatgagtcagtcttttctgcaccttgattcagtccaaagccatctctgttaatattgatggaaacagaacctgtgactcgatgccaccgtcgaaccaaaaatttcattctggaaattgcaatggatactctgacggccgaccgaaacctggtgaagccctttgggcgattggtgatcacctctagatccgtgaaagctggctgcccccccatccgggcaagcagggccaaggtggcatcttcacattcctggaacccacccagtaacagcagcaggtatttcttctggtaaatgagagcctttcgaaaactttctgccctcaagtatttaccataaattctctttaaagtgacatgttcagaatcagggctcagagtttgaagtaaagagtcatttcttagttcagctttcagtttgtatacttcagcctctgcccttttcaaagatttctggagagtcaatttttctctgttccatacttctttttcagaggcaatgatggcttcaatgttggcaccaccattcaatgaaaacctggaagaattatctctaccagctcctgtctgtcgataccacctgatctgctcttccagcttcataaccatgttccttaagtcattcttctcttcagtcagttgactgatatgccctgtcagctcagcattttgtctcagtagtctttcagtcaatgagccacaagaagtacttggggacaccaagctgggctcttcaccttgctggccagttaatttctgtagttgtaaaataatttcatcaatattttcctgaacccaaatgaaatcttcatcatctgctgtttcaaactgtagtctctcagaggctttctggggtagaacctgtagttttgaagctacacattgaagcttttgtctgatcatttctaattcatgattacagccggttcctcctccattcatttcaatcaatttagcgtagtttgattcttttgtttctccttctattttctgttgaagaacccaatttctagttctatcactggttaagctccacgtggttggctcattaaggttctgatacagaattcttctactttctcgtttttcttctcgttctagttcttgcttctggaattcctgcatgattccttgtagtcgctgtccttcaaggtctaacttataaacttgttgtcttttctcttccagctggcgctgaagatcttccactttggactggagctcatgcatttttttctgtccctcagtgttggcctcctgttctgtctgcagtgttttcctgtgaacctgcctatctttttccatttgctgtcgtgtttgcaaagaatccagtttatatttttcagtctcatttaacaattctactatgcgactgtgtttttcctctagctgtttctgcagctctttcagtaggtcctctgagggcaagggtggccgagactgtccagtaccatcactgctctgcagctgtgcgtgcaattcccgctccctatctagggtactactcatttcccgaattcgaactttctcagattcaagaagtacctgaagctctaagtttcgaccttgttcttctgacaactgggcatcatatagcattctctgtgattctattttttgctgggattcgttcagtagttgtttctgttgttccaaaagtagatttagctgaagattcctttgtttctgactctcaagtgaaaacttcagatcctcaagttcttctttatcccgttcttcactgcgtcccaacttggctttctctttctccaaagcccactggagctctcttgattttttctgttcacttgctaatgtgtcattaagcaaatgtacttcatctgtcttatctttaacttccaacctgaaagcctccaattcttttaggtgtttatgctgtgccttgagtgttgtttctagttccaatttagtttgtgcaagctcactcttcagttcagcaaccaccattttctcagaactcagctgctcctgcagttccgttgctctgtctttcatactgctgagctccacttgcatctccagcatttgagactgcttctgctgtatattatattccaagagttcttggcttggtttctcactctcttgttctcttttcagagtaattttcctaccattcatttgtgcatgcagtgcctgaatttcagataacaaactccttctatctgctttctggaggcattccatagctgcttgatattcaacaccctgttcttgtattctctgttccaaacagtttagtaaaccaactgcatctgtagtacctagagctgtcagctccgtccgaaatgctgctagtaaaacactacgctcttctaagaaaacttgttgaagggcaagcagtagttcacctcgccagtctgagaagctctcatgagattgagaactatcataaacctcggcttctctttgcagttgcatctttgtaattaaatcctttagagatgagattgtattgatgtaagcttttctctcttctagccaaggttctgaaacctgctgaatagaatggtcctctccatcactatagggagactcagtgagagaaagcacctgcatgccttcattatggacagctctcagtaatccctttattttctttggaaaggaatctgttgcactttcactttcttctcctcggccttctgatgctatgtcaaatccctgactgtgtgtaagataaattccctgaccccagtctgatccagaatcactggagcatatttctctagtctggtaagcatcagaatgtgctagctcaggaattgaggatccctctttacttctcagacactgtatcactgccttcaaggtaccacattcctctttcagtaactgaacggcaacatagtgttccctctttaaggtttcagtttctgaaatatgtctggattccatgtccaaaatttcagcagcatgtagttcttgcatcttctcaattttttcagtaaactgactgattatttcagtaacttcttctgaggaacattcactctgtaaattaatttgtattcctgcatttttaacaagaatttgtggagtctgattgctgctactgatcttcagagtcccatctgtctgggatgcaatgctcttactcagttttataggaagtggctcaaacatgcaggcctttttgctttcttgtacctcagtctcatcttctttttctaaaatggacaatttctcttttgcctctgcgaggtgatccctaacttggcttaagtctttctgaagagatgtcatatttgtttcttttaccaaaagctcttcttgaagtttttcagccttttctttataactggcaagttctgctttggtagccactgattcagctctaagagcctcgagttcattaaaaaatccactttcttcattgctatgaaatagctcagtagttgtcttgagaacttcaacatcttgagggcttcttttcttttctttctctctctgttttttctcattgccctccaatagcttctgtagttctagcagcttcttttctttttctaaaacatttttttctgcaatttctacttgttctttttctaaaatcaaactagtatgcatttcaacaacctggctttctaattctgatattctcaaggttaatgctgatatatctgaccccaactcatcttctcttagttgatttaaattctgaatatttgttctttcaggttctgatgaaattgtttgattatcttgacagaattttgcatattcctgaactgcctcaagttggatttgactgacaagagcagcagccactttttcttcaactattttctgtaggtttacaatcttcttttgaagcatttctgtttcaaactggccttgttcttgcatgtcttttatttgtttataacactgggtaagttctaagtcctttgcactaacagtgctctcaagttgtagcaaccttgtttccaaattaattatggaacctttgccattttcttcaaaagatttgaagtatgtctgattttctagggatttaagagcatcctctgtaaggactacttctagttcaggtttgtctttgctcagatgatctatagccacgttaacactattctctggtatgctttgaatcttttccacactttcacgttctctctttaagctgaataattcctgtgttagctgattcattttaaaattggtttctttaagtacatttttcatgaaggtcatttcttcattagcggtttctacttgctgttccaaggccagcttttcagctataaccacatccaattgatgttttaaactgtctgcttcttctgagagggaatgagcattcattgatgtcttctgtccaatatttgccaattcctgttgaagtttttcaatcacttcattgagctgctctatttcttcttctctatttctcttcacacattcttgatcactcatcaaacattctatttgggtttcaagatcccttatcagttcatttttttcttcaataaccttgttatctgttgtaattttaagttgctgctggagtttcgtaacttgttcatttaattggtcaatttctacctctttttcctgtattatttgagcaaatttcccaaatagcacatgttggtcttgagtagacatggcatcagattcctttatggcaagtcccagtttctccatgtcatccttaaataatttgttttcctgttcaagttcttgtaggcgggtagtagattcctttttctgtatttctaattgcatatgtaattgttgaacttcttcattcttattttccagttcttctctaaactgttctaattgctcttctaagtttgtaatctctttttcctttctgtctatggcatctcgttcagcctgcaattgtacttctagggacaattctggtttagcttctacagctccaaagtgttttcggtcctctaccttttgaaaagtatctgcactcacaagaagcgcctgctccagttctcttactctgaactccagtttctctatttcttcattcctttcttgtatatccctttgaagctgctctttagagagcaaaagctcactgcatttgtctgttttttctttcagatgatttgctaactgttcaacctctctagtttgatgttcactgataggctggaatcgaggaacaaccttaagttgctgttctagtttctgtatttcctgttggaatacatctctctcatgttctctgtcaatggcttgctcatctaaaaattttctcattttttctaactgcttttccaatgcttggttttgctgtcttaaatccattagttcagtatttttttcttgttccagctctataaacctactgacttgttcttccacatctatttctagagctttcacttgtttttgaaggtcatcacgtactttttcagcttgacattgtacttctagtttttccttcattaatttttctgtctcctgtagtaattgttgttcaactgggcctgcctctgctttcatagcttccttttgtctggacagtaattctctttcttcttggatctgctgttgctctgcctccaattcttgcaacctgttacttgcacataacaactcctgctcaagacgatctattatatcagttttttcctgaatttgcctttcaaaaagagttttttcatctgcatagccatcaatgacgccctcagccttactgagctccacagctagctgttctctggccctggactcctcatgaaggcgctctcgaagttcctcttggcacttaagggactctgttgcttcttgtttctgtctaaatgactcacgcatcaactctgtctgtgtcactttcgcatgttcaagtgaataaggaggggtaggcagtgaaattttagaaataagctttaatatatgcccgtttcttttatgaataaaatggaaaatagaagtattaacaattactgagttattttcatccaaatgttcacaaagaggaaaaggatgtggtaaaggcacgcgagattcaacctcataaatgtcttcatcttgctcttctaaccacgagccactgactttgacagttgccaaataggtgctataagaatccatcccagaagatacagctgccgagattcctaatttgctttatcaattttctaatacattaaaaagttctttttagtttatcaagatctaccatagcagtataaaaagtttcttttttagcactatcaaataaatgttataaaattaattcatacaactgcacaataaaaggaaggggaaagtccaggaaaaaaactacaaatctaaaaaaacttaggtctctatcaatcttgatgccccctcaaaaaaacccaaaccaaaacaaaaaccaaaaaaaatcaaaaaacaaaaataaaagcaagcaaacaaaaacaccttttaaactagcataattaagtccttgaagagaagaataaaaatataaacatctaattagacgagcaataaaactgcttttaatatcagcgatgtctgtagtaataagtaagccttcaaagcagaacctggcagggaaggtcaagtttgaaatctccatagcagcagtcttgagaaatgcagttgtaacattatttctcttgctcttgctgcttcactctattcaaaaggaaaagctcttct

SEQ ID NO: 14141 - RNA, 14452 nt, Homo sapiens
  source 1..14452: mol_type = other RNA
gctgggattacaggcatgagccaccgcacctggccttccctgcttcctctctagaatccaattagggatgtttgttactactcatattgattaaaacagttaacaaacttttttctttttaaaatgtgagatcagtgaactctggttttaagataatctgaaacaaggtccttgggagtaataaaattggtcacattctgtaaagcacattctgtttaggaatcaacttatctcaaattgtaactcggggcctaactatatgagatggctgaaaaaataccacatcgtctgttttcactaggtgatgccaaaatattttgctttatgtatattacagttctttttaaaacactggaagactcatgttaaactctaattgtgaaggcagaatctctgctaatttttcagattaaaattctctttgaaaaaatacagtctgtattcatgaattgtaaaatatgtgcttcagtgagcagagttagggaatccaggaacttgggtggggaaaaattacatctttatttgcactaataatttctaactgcaatttagtatttatttcaattatgaatttgggcagcattttattagcagtatccatgattttgtcaatagaaatctcagatattttcatattacagatgttacagatttcttgaagtatctagttacgaccccgagataaggctagtctaatgtttagtgaatagttttagacttcttaacagatttcatttttaatcacagactaattaattattgagatgcataaacaagtgtgattgcagaggcctactatcataaggaggcgtggtggtcaaacaatggcactgaactcagcttgatcagatcatttgtccatctgtttttttctccactgtctcttagagcagaatagccttgaatggcaagccatgctagctgaaaaaggtttttacccacaacctgccccttcaactaactgctttagagtacgtttgctatttttagaattcctcttattggaacccagcttctaatgtggaaaatttaagtatagttggctccttttatttgtgggttctgtatcctctgattcaaccaactgcaggttcaaaatactaaaaataaaaccccacaataaaaaaatacagtattagcaactatttacataatgttcacattgtattaggtatcaaataatctggagatgatttgaagtacacaggaggatgtatgtagactatctgcaaatagcacattgttttataagagacttaagcattcgcggactgtaatatccaagggggatcctggaactaatcccccacacatgccgagggatgactgaaattagaaatgttcaagcatgtacaactttctaccatgcctgtttgtgttggtataaatcatggaacatcaaataataagacaaaatcctccaggtgtaagcatcaaatactagtcctcttgctgttttagtgagttgccatgttattgaggaggactccagatgagaaataacattgcgatctgtattatctctgtgagagcctcccagtctgaatttggcttggacaacagggatactgtttaattcggctgcaatgtgattaagatcttttgagttaatgatttcttcatctttttagtgggccatggatttgtgagaacacatctttggaaacaagtaacactaactgtaatatagtaaatactgattaatcatgaaataccaatatagcttttaaaaaacactatgtagatgtaaagttgatacaaagacacatggaaaactttcaacagtattaactctaagattaggacaactttctctgaatctctcactcctacatatttgacataagtaatgagatgctatgtaccaagaactatggctcagttaaaaatgaagaaggttcaaatacagtgtggtgaaaatggtgaagtcatttttatttcagtacttgacaaaataccccataaaattcaaaacttctaccattatacaaaaataggtctctacaagtgatattatctgtcttcatcaccagtagaatatattaggcaaaacatgtaacttcagtagccttataagaaaagtgcaggacacctcgagctacacattcagcagtattgtaatgcgtaaaagtttaatcttttcacccatttgataaatacacaaggtttataatttaatgttttaaattagcattccacaaatatacaggtaattcaataattattgtgcatgaatacatacacaatgcttatatatacaaattccagtttgttttcatgtgctggcaagggatttgtatacaatcataagctgtgttcatattggtcccattgaatattcacaatacaaaagcacaaaagaaccattgatttacaaaaggaaatctatttaaaatcacttcaattaatgatgtttcaaaggattatcttctcatgccagcatgaaattgagtagttgaacctgactgtatagttccaagtcgtctttgcagtgcctctagccgagtgatataatctgttagggctctgtcaggatcgtaattctgaagctgagaacatgctaaagaaccaggattgaaatcagctggagtgcctgggtacctattctgaaatggtaaaggggacctaatatagtccagatctgatcttgagcgatacgtagtatgtcttggttctccatataactccagcccaccagaagaatgataaaatgagtcagtcttttctgcaccttgattcagtccaaagccatctctgttaatattgatggaaacagaacctgtgactcgatgccaccgtcgaaccaaaaatttcattctggaaattgcaatggatactctgacggccgaccgaaacctggtgaagccctttgggcgattggtgatcacctctagatccgtgaaagctggctgcccccccatccgggcaagcagggccaaggtggcatcttcacattcctggaacccacccagtaacagcagcaggtatttcttctggtaaatgagagcctttcgaaaactttctgccctcaagtatttaccataaattctctttaaagtgacatgttcagaatcagggctcagagtttgaagtaaagagtcatttcttagttcagctttcagtttgtatacttcagcctctgcccttttcaaagatttctggagagtcaatttttctctgttccatacttctttttcagaggcaatgatggcttcaatgttggcaccaccattcaatgaaaacctggaagaattatctctaccagctcctgtctgtcgataccacctgatctgctcttccagcttcataaccatgttccttaagtcattcttctcttcagtcagttgactgatatgccctgtcagctcagcattttgtctcagtagtctttcagtcaatgagccacaagaagtacttggggacaccaagctgggctcttcaccttgctggccagttaatttctgtagttgtaaaataatttcatcaatattttcctgaacccaaatgaaatcttcatcatctgctgtttcaaactgtagtctctcagaggctttctggggtagaacctgtagttttgaagctacacattgaagcttttgtctgatcatttctaattcatgattacagccggttcctcctccattcatttcaatcaatttagcgtagtttgattcttttgtttctccttctattttctgttgaagaacccaatttctagttctatcactggttaagctccacgtggttggctcattaaggttctgatacagaattcttctactttctcgtttttcttctcgttctagttcttgcttctggaattcctgcatgattccttgtagtcgctgtccttcaaggtctaacttataaacttgttgtcttttctcttccagctggcgctgaagatcttccactttggactggagctcatgcatttttttctgtccctcagtgttggcctcctgttctgtctgcagtgttttcctgtgaacctgcctatctttttccatttgctgtcgtgtttgcaaagaatccagtttatatttttcagtctcatttaacaattctactatgcgactgtgtttttcctctagctgtttctgcagctctttcagtaggtcctctgagggcaagggtggccgagactgtccagtaccatcactgctctgcagctgtgcgtgcaattcccgctccctatctagggtactactcatttcccgaattcgaactttctcagattcaagaagtacctgaagctctaagtttcgaccttgttcttctgacaactgggcatcatatagcattctctgtgattctattttttgctgggattcgttcagtagttgtttctgttgttccaaaagtagatttagctgaagattcctttgtttctgactctcaagtgaaaacttcagatcctcaagttcttctttatcccgttcttcactgcgtcccaacttggctttctctttctccaaagcccactggagctctcttgattttttctgttcacttgctaatgtgtcattaagcaaatgtacttcatctgtcttatctttaacttccaacctgaaagcctccaattcttttaggtgtttatgctgtgccttgagtgttgtttctagttccaatttagtttgtgcaagctcactcttcagttcagcaaccaccattttctcagaactcagctgctcctgcagttccgttgctctgtctttcatactgctgagctccacttgcatctccagcatttgagactgcttctgctgtatattatattccaagagttcttggcttggtttctcactctcttgttctcttttcagagtaattttcctaccattcatttgtgcatgcagtgcctgaatttcagataacaaactccttctatctgctttctggaggcattccatagctgcttgatattcaacaccctgttcttgtattctctgttccaaacagtttagtaaaccaactgcatctgtagtacctagagctgtcagctccgtccgaaatgctgctagtaaaacactacgctcttctaagaaaacttgttgaagggcaagcagtagttcacctcgccagtctgagaagctctcatgagattgagaactatcataaacctcggcttctctttgcagttgcatctttgtaattaaatcctttagagatgagattgtattgatgtaagcttttctctcttctagccaaggttctgaaacctgctgaatagaatggtcctctccatcactatagggagactcagtgagagaaagcacctgcatgccttcattatggacagctctcagtaatccctttattttctttggaaaggaatctgttgcactttcactttcttctcctcggccttctgatgctatgtcaaatccctgactgtgtgtaagataaattccctgaccccagtctgatccagaatcactggagcatatttctctagtctggtaagcatcagaatgtgctagctcaggaattgaggatccctctttacttctcagacactgtatcactgccttcaaggtaccacattcctctttcagtaactgaacggcaacatagtgttccctctttaaggtttcagtttctgaaatatgtctggattccatgtccaaaatttcagcagcatgtagttcttgcatcttctcaattttttcagtaaactgactgattatttcagtaacttcttctgaggaacattcactctgtaaattaatttgtattcctgcatttttaacaagaatttgtggagtctgattgctgctactgatcttcagagtcccatctgtctgggatgcaatgctcttactcagttttataggaagtggctcaaacatgcaggcctttttgctttcttgtacctcagtctcatcttctttttctaaaatggacaatttctcttttgcctctgcgaggtgatccctaacttggcttaagtctttctgaagagatgtcatatttgtttcttttaccaaaagctcttcttgaagtttttcagccttttctttataactggcaagttctgctttggtagccactgattcagctctaagagcctcgagttcattaaaaaatccactttcttcattgctatgaaatagctcagtagttgtcttgagaacttcaacatcttgagggcttcttttcttttctttctctctctgttttttctcattgccctccaatagcttctgtagttctagcagcttcttttctttttctaaaacatttttttctgcaatttctacttgttctttttctaaaatcaaactagtatgcatttcaacaacctggctttctaattctgatattctcaaggttaatgctgatatatctgaccccaactcatcttctcttagttgatttaaattctgaatatttgttctttcaggttctgatgaaattgtttgattatcttgacagaattttgcatattcctgaactgcctcaagttggatttgactgacaagagcagcagccactttttcttcaactattttctgtaggtttacaatcttcttttgaagcatttctgtttcaaactggccttgttcttgcatgtcttttatttgtttataacactgggtaagttctaagtcctttgcactaacagtgctctcaagttgtagcaaccttgtttccaaattaattatggaacctttgccattttcttcaaaagatttgaagtatgtctgattttctagggatttaagagcatcctctgtaaggactacttctagttcaggtttgtctttgctcagatgatctatagccacgttaacactattctctggtatgctttgaatcttttccacactttcacgttctctctttaagctgaataattcctgtgttagctgattcattttaaaattggtttctttaagtacatttttcatgaaggtcatttcttcattagcggtttctacttgctgttccaaggccagcttttcagctataaccacatccaattgatgttttaaactgtctgcttcttctgagagggaatgagcattcattgatgtcttctgtccaatatttgccaattcctgttgaagtttttcaatcacttcattgagctgctctatttcttcttctctatttctcttcacacattcttgatcactcatcaaacattctatttgggtttcaagatcccttatcagttcatttttttcttcaataaccttgttatctgttgtaattttaagttgctgctggagtttcgtaacttgttcatttaattggtcaatttctacctctttttcctgtattatttgagcaaatttcccaaatagcacatgttggtcttgagtagacatggcatcagattcctttatggcaagtcccagtttctccatgtcatccttaaataatttgttttcctgttcaagttcttgtaggcgggtagtagattcctttttctgtatttctaattgcatatgtaattgttgaacttcttcattcttattttccagttcttctctaaactgttctaattgctcttctaagtttgtaatctctttttcctttctgtctatggcatctcgttcagcctgcaattgtacttctagggacaattctggtttagcttctacagctccaaagtgttttcggtcctctacaagaagcgcctgctccagttctcttactctgaactccagtttctctatttcttcattcctttcttgtatatccctttgaagctgctctttagagagcaaaagctcactgcatttgtctgttttttctttcagatgatttgctaactgttcaacctctctagtttgatgttcactgataggctggaatcgaggaacaaccttaagttgctgttctagtttctgtatttcctgttggaatacatctctctcatgttctctgtcaatggcttgctcatctaaaaattttctcattttttctaactgcttttccaatgcttggttttgctgtcttaaatccattagttcagtatttttttcttgttccagctctataaacctactgacttgttcttccacatctatttctagagctttcacttgtttttgaaggtcatcacgtactttttcagcttgacattgtacttctagtttttccttcattaatttttctgtctcctgtagtaattgttgttcaactgggcctgcctctgctttcatagcttccttttgtctggacagtaattctctttcttcttggatctgctgttgctctgcctccaattcttgcaacctgttacttgcacataacaactcctgctcaagacgatctattatatcagttttttcctgaatttgcctttcaaaaagagttttttcatctgcatagccatcaatgacgccctcagccttactgagctccacagctagctgttctctggccctggactcctcatgaaggcgctctcgaagttcctcttggcacttaagggactctgttgcttcttgtttctgtctaaatgactcacgcatcaactctgtctgtgtcactttcgcatgttcaagctgactgctagtttcacttatggcttctaggagtttttcaactgctgcttgtagtcgagagctaatgttcagcataagttcttcattttcagggtctatttcagttccagcaaaaccactcctcacaagtcgttgtgacagctctgttccttcctcagttacttttgaccacatgttaatgtcatttcttggcatatcacttccagaataagagggaatggattcatctgtaactcttgtatgttcctcatggacacatgactttacagatgcctctgcttctgacctccaaattaggctggcagatgactggcttttactagatctatctagaatcccaaggacatggcgaccaattgtttcttcaacagctgctgttgtctttacaacttctaagaggatcttcaaaagtctattattagctttctggagtgcatacactgtctttcttgtttgagttccatactgactgcgttccatactgatgatccaatggggaagccaaaatcttaggggccaaattcctccatgcaagctttcattagacaaaatctcaggaggcacatcttcaggttttctgtctaattccttttctttaaatgtttgttcttcaacttctccttggttttcatttccattctgtgtttgcgtactgctgttgcgcagctcacaacacagcttctctcttccagctaaagacagctgctttagtgcttccagctcctctaaaagcaccctctctctctctgaaaccaggttttcattatctatggaggatctctgggctaattgtctattaagtctcttaatctcttcttgtagctgttcctggtcttctcgctgtctctccatttgccgcatatgtgcttgccttaacaattccgttgcctgttgatgttcttggtattgtcgtacaagttcctgtctcatatcttccaactgttcttcattcaacattagttgtctagaagcatccatgcttgacactgaaatctcatcatgaatagactgtctaactataaatgttttatctttggagaacatttcttctgaaatagtcagcacacagtcctttgattctggtatatcatggggatcactatttgataataaaatttcctttccatgttctcctaactctttactaagtggtttaaattcttctttaaatttcacatccactgtctcaaaagtctgaaaaccaatttgatcctgtgataatttcatttcattaaaataatgttgttcttgctgacacacagcatgtgcttgctttgatgatgcagtattttcttttcccccagatattctagacagttcagtttgttgagcaaatgctatactcattgacacaataaccttagctacttcttcttctaattgttcttggtattgtttttcaagcaacttaacgatatttgtttcctctttcactccaaattcaccagaaaactctattgtaccatcaatattctttttcacacaacttccagggtacattgttctctgtgcatcagattctgtaattaccaccgaatcaacaggtaagcttggcggaaccgtggactcactaacagcttgaagcctcttctgtaaacagtggatctctgcctcatagttttgttcagtttctttcaactgttgctgcaaagaggatatgaggctttctaattcttgaacttgttcttcaagtttagttttttcaagatcttgcagagaagataacttgcttttatgattgacatcaatgtcttccaaattggtcatctgagaatggattgataaaaactctgtttcctcttttggaaggttttcttctccaaattcaagtttcataccatctgtctgctgtccccagatcttgcttagtcgtgtttgaagtaccaagagtttgttgtattcttctgttactttgttgagaagagtgtgcatattttcttgaaagtcttgaacttcatatctataatcttgtaattctggatcttcattttcagaaatgtaatcaccagaattctctttgtcttctgcatttacttcacattttaaagcaggagtataatattcaccaaggacactgcataaagtctgtaaaaaataagaacattcttcagacactgccttttgaagttttccaatgagcagatgtaaaggctttccttcatcacctgtttcttgtgttttcatagtctgtagttctaactggtgtattttctgaagttccttgatcttttcctcttgagcaaaaataagctcttctttaagactgcaaagagctttatctttttcattttccatatattcacgaacctgatccacatgagttgaataaaccagagagaggcaaatgcgttgggcttccatctgtagccttaaatcattctgttctgatttaagtacattgagttctttctgaagtttatcattttcacttggttgagttgctctaagtgatgattcctttgttacagatggtaagtgatccaaaatcaactgttcttgcttactttcttctccaacagtcatattttcaaaagaaactttatcttccaccattatttttgattcttcaccaaaacttttatttactttagaaactgatccttcagcacccctgcttgtcatggtcacaactccatctaataaagagcttacttgagtatcacatgactgtacattttctgccctgttgtggttaataatgatttctagctctctacatctcaatgaaacttgttctttctcttgctttaaagatttaacttcttcatttagaaaactaatctcaccatgtttctgtttcaattgttcagaaagatcagacagtctctgtgacagctctaatttctctcgcttggttacctcaagtttttccatgagttctgttgtatccttttcaacaacctcacccatttccaatgtttctgctacaaaagttttgtcttcatcaaagacagaacttttcattttcactgtagttggatttattctttgcaaatgaagctcttcattaagtgctttaagtttacttttatactctaattcctgtttatttttactgtcttctaaatcatcttttactttgagaaggcaagcatactcctcttgtaactcttgatagttaacttcaaagtttttttcagcaaatgaaaaagtgttcctttgcttttcaatctcttcatttagctgaatacattgttgtttgaggtcctcattttcctctataagtatttctatttctttttcccacacagagtctttggatttggacttaatggagtctaagaaaatcaatctttcttcttggctaacaggagtatgtattttcaacatgtcttcaagggttttcttttcatctttaagaatgctattctctgcttcaagttgtgcaaatttttcttgaagatcattctctttttccttcatctgtttttctaacaattctgttttaagttgtaattcttgaacttcttgttcaagtgtacccttttctttttcttcttgtctgagtatttcaatttctttttgaagttcattgatttgaagagtcatttcttctgactttgaatttacaagagactgctgtaaatcttttagctttgaaatttccaaaattaattgattctgcttagttatcaaattgtccttttcaaactgcatggtttctatcttttgactcatttcattctgtaaaccatctatctgctgtttatagtgaatgcctaaattatctttaagtttttcaatatttattcgatgttcaatttctaaatcttccttcagtttggaaagctcttcttcgtgactaaatagaagctgtgttctcagcctctctaattcagcttcttgtgattcagccattctgtctaacacagcattcttttctttttctaacatttcaagttttatcttgtaatttgtaacttctgcttcatgttttaattctagttcctttctggattcagatgcagaaacaatctcagctttcaaatcttccactgtactaagggacttatgtgcttcattaagtttactttcttgttcagctattgtctgtctagctctctgaatctgttcccttgaaaagctcaattcttcaacaaggtcttcaagctgtctctgtagagcacacttttcttctaaaattagtcctagttcttccttgagtttttccttttgagagttagtatcttgcaattttatattcagttcatttattgccacattcattaactttatctgatcttcattaactgtaatatttgaatatgaccttaaagcattctccatttctcccttatgccgtgttttcatttcctccatctgtgccatgtgttgtcttattaattcttgtttcatttgcactatctgctgcccatacatctcatccagctctgcccggagttgttctaactttctttgtgtttcttgttccattcgttgtactatatcagtttcgaactggctgtctttatgatttctcttctgaagttcttcgactgtccccattaactgttttatttcttcagaagactgtctttctttttgcttagaattagtcagctctaatttcatgttttttatttcttggttcttttgcacaatctgttcttgtaattctcctagtaatttatcagcagttgttaatttatcctttagctcaagagttttcttttcttcttctattatttttgtgtttaattcttcaatgattgtctccttttcctgtatttcttctttatttgagttttctacttttttatcttgttccatttcatatactttaattttctcttgcaagaaactaatttgcattgtgaagtcttctttctttttctgataatcttctaataagtggtcttgttcttcaagctgctgttgatgagtgaggatctgttgtttggcttgtagtaagtctgcagctgtgctactatgagtgctgtttctcagagtttcactagcctgtaattgctgaaattgaatctgtaatttttgactctgttctgtcaactctaaaaattctctcattgtctcatccttttctcttcttgcttgttgtaaattagcagtgagctgggttataatgccatctctttgtttaatggcagcttcaaattcttgtaactgctgcagtccttcagtcccataggtaaccctcatttcttccagctctctgtttagctcttcaatctcatgctgcttcccagccaactcactttccatcatctctagatgagtcggactgtcttgtgctccttgttcagaataagaatcatcaacaccaaattcttcttcccttaataaatttgtaggctttcctgttctcatcacaaaactgcaaccatttacctctgaactgcagtcatctgctgtggttgaaatttcactttccagttccacagagaagccctgctcatgactggttatttctccactatgtagagttctcattattgtagattcaggaatcacagttgattctactctctgagaactatttatgtacatttcattacactgtgattgatcaatattcaaatcatggtgtgctgacacatcatgtttactgcttgacgtttttctcttttttttctgcttcttggaaggactctgcccatccgactgagcttttctttgtcgaaactgggcaagcttggctttgccggcctccagcttcttctgtctctcctcgtcctccatggcctctgcaaggaaggcaggggaaaacaggggttgaggggtggttggggatagaaaggaaaggtcgatttggacggaggtgggacggcaagctccacggcctagagagccgattcggtccggcgctcccccgcccgaagtggaagcagtctccgcgctcactggcggatcgtcctcagccgcacgggaagcgccgtcaccgccgccgccgccgccatcttcgtctccacgta

SEQ ID NO: 14142 - RNA, 14515 nt, Homo sapiens
  source 1..14515: mol_type = other RNA
gctgggattacaggcatgagccaccgcacctggccttccctgcttcctctctagaatccaattagggatgtttgttactactcatattgattaaaacagttaacaaacttttttctttttaaaatgtgagatcagtgaactctggttttaagataatctgaaacaaggtccttgggagtaataaaattggtcacattctgtaaagcacattctgtttaggaatcaacttatctcaaattgtaactcggggcctaactatatgagatggctgaaaaaataccacatcgtctgttttcactaggtgatgccaaaatattttgctttatgtatattacagttctttttaaaacactggaagactcatgttaaactctaattgtgaaggcagaatctctgctaatttttcagattaaaattctctttgaaaaaatacagtctgtattcatgaattgtaaaatatgtgcttcagtgagcagagttagggaatccaggaacttgggtggggaaaaattacatctttatttgcactaataatttctaactgcaatttagtatttatttcaattatgaatttgggcagcattttattagcagtatccatgattttgtcaatagaaatctcagatattttcatattacagatgttacagatttcttgaagtatctagttacgaccccgagataaggctagtctaatgtttagtgaatagttttagacttcttaacagatttcatttttaatcacagactaattaattattgagatgcataaacaagtgtgattgcagaggcctactatcataaggaggcgtggtggtcaaacaatggcactgaactcagcttgatcagatcatttgtccatctgtttttttctccactgtctcttagagcagaatagccttgaatggcaagccatgctagctgaaaaaggtttttacccacaacctgccccttcaactaactgctttagagtacgtttgctatttttagaattcctcttattggaacccagcttctaatgtggaaaatttaagtatagttggctccttttatttgtgggttctgtatcctctgattcaaccaactgcaggttcaaaatactaaaaataaaaccccacaataaaaaaatacagtattagcaactatttacataatgttcacattgtattaggtatcaaataatctggagatgatttgaagtacacaggaggatgtatgtagactatctgcaaatagcacattgttttataagagacttaagcattcgcggactgtaatatccaagggggatcctggaactaatcccccacacatgccgagggatgactgaaattagaaatgttcaagcatgtacaactttctaccatgcctgtttgtgttggtataaatcatggaacatcaaataataagacaaaatcctccaggtgtaagcatcaaatactagtcctcttgctgttttagtgagttgccatgttattgaggaggactccagatgagaaataacattgcgatctgtattatctctgtgagagcctcccagtctgaatttggcttggacaacagggatactgtttaattcggctgcaatgtgattaagatcttttgagttaatgatttcttcatctttttagtgggccatggatttgtgagaacacatctttggaaacaagtaacactaactgtaatatagtaaatactgattaatcatgaaataccaatatagcttttaaaaaacactatgtagatgtaaagttgatacaaagacacatggaaaactttcaacagtattaactctaagattaggacaactttctctgaatctctcactcctacatatttgacataagtaatgagatgctatgtaccaagaactatggctcagttaaaaatgaagaaggttcaaatacagtgtggtgaaaatggtgaagtcatttttatttcagtacttgacaaaataccccataaaattcaaaacttctaccattatacaaaaataggtctctacaagtgatattatctgtcttcatcaccagtagaatatattaggcaaaacatgtaacttcagtagccttataagaaaagtgcaggacacctcgagctacacattcagcagtattgtaatgcgtaaaagtttaatcttttcacccatttgataaatacacaaggtttataatttaatgttttaaattagcattccacaaatatacaggtaattcaataattattgtgcatgaatacatacacaatgcttatatatacaaattccagtttgttttcatgtgctggcaagggatttgtatacaatcataagctgtgttcatattggtcccattgaatattcacaatacaaaagcacaaaagaaccattgatttacaaaaggaaatctatttaaaatcacttcaattaatgatgtttcaaaggattatcttctcatgccagcatgaaattgagtagttgaacctgactgtatagttccaagtcgtctttgcagtgcctctagccgagtgatataatctgttagggctctgtcaggatcgtaattctgaagctgagaacatgctaaagaaccaggattgaaatcagctggagtgcctgggtacctattctgaaatggtaaaggggacctaatatagtccagatctgatcttgagcgatacgtagtatgtcttggttctccatataactccagcccaccagaagaatgataaaatgagtcagtcttttctgcaccttgattcagtccaaagccatctctgttaatattgatggaaacagaacctgtgactcgatgccaccgtcgaaccaaaaatttcattctggaaattgcaatggatactctgacggccgaccgaaacctggtgaagccctttgggcgattggtgatcacctctagatccgtgaaagctggctgcccccccatccgggcaagcagggccaaggtggcatcttcacattcctggaacccacccagtaacagcagcaggtatttcttctggtaaatgagagcctttcgaaaactttctgccctcaagtatttaccataaattctctttaaagtgacatgttcagaatcagggctcagagtttgaagtaaagagtcatttcttagttcagctttcagtttgtatacttcagcctctgcccttttcaaagatttctggagagtcaatttttctctgttccatacttctttttcagaggcaatgatggcttcaatgttggcaccaccattcaatgaaaacctggaagaattatctctaccagctcctgtctgtcgataccacctgatctgctcttccagcttcataaccatgttccttaagtcattcttctcttcagtcagttgactgatatgccctgtcagctcagcattttgtctcagtagtctttcagtcaatgagccacaagaagtacttggggacaccaagctgggctcttcaccttgctggccagttaatttctgtagttgtaaaataatttcatcaatattttcctgaacccaaatgaaatcttcatcatctgctgtttcaaactgtagtctctcagaggctttctggggtagaacctgtagttttgaagctacacattgaagcttttgtctgatcatttctaattcatgattacagccggttcctcctccattcatttcaatcaatttagcgtagtttgattcttttgtttctccttctattttctgttgaagaacccaatttctagttctatcactggttaagctccacgtggttggctcattaaggttctgatacagaattcttctactttctcgtttttcttctcgttctagttcttgcttctggaattcctgcatgattccttgtagtcgctgtccttcaaggtctaacttataaacttgttgtcttttctcttccagctggcgctgaagatcttccactttggactggagctcatgcatttttttctgtccctcagtgttggcctcctgttctgtctgcagtgttttcctgtgaacctgcctatctttttccatttgctgtcgtgtttgcaaagaatccagtttatatttttcagtctcatttaacaattctactatgcgactgtgtttttcctctagctgtttctgcagctctttcagtaggtcctctgagggcaagggtggccgagactgtccagtaccatcactgctctgcagctgtgcgtgcaattcccgctccctatctagggtactactcatttcccgaattcgaactttctcagattcaagaagtacctgaagctctaagtttcgaccttgttcttctgacaactgggcatcatatagcattctctgtgattctattttttgctgggattcgttcagtagttgtttctgttgttccaaaagtagatttagctgaagattcctttgtttctgactctcaagtgaaaacttcagatcctcaagttcttctttatcccgttcttcactgcgtcccaacttggctttctctttctccaaagcccactggagctctcttgattttttctgttcacttgctaatgtgtcattaagcaaatgtacttcatctgtcttatctttaacttccaacctgaaagcctccaattcttttaggtgtttatgctgtgccttgagtgttgtttctagttccaatttagtttgtgcaagctcactcttcagttcagcaaccaccattttctcagaactcagctgctcctgcagttccgttgctctgtctttcatactgctgagctccacttgcatctccagcatttgagactgcttctgctgtatattatattccaagagttcttggcttggtttctcactctcttgttctcttttcagagtaattttcctaccattcatttgtgcatgcagtgcctgaatttcagataacaaactccttctatctgctttctggaggcattccatagctgcttgatattcaacaccctgttcttgtattctctgttccaaacagtttagtaaaccaactgcatctgtagtacctagagctgtcagctccgtccgaaatgctgctagtaaaacactacgctcttctaagaaaacttgttgaagggcaagcagtagttcacctcgccagtctgagaagctctcatgagattgagaactatcataaacctcggcttctctttgcagttgcatctttgtaattaaatcctttagagatgagattgtattgatgtaagcttttctctcttctagccaaggttctgaaacctgctgaatagaatggtcctctccatcactatagggagactcagtgagagaaagcacctgcatgccttcattatggacagctctcagtaatccctttattttctttggaaaggaatctgttgcactttcactttcttctcctcggccttctgatgctatgtcaaatccctgactgtgtgtaagataaattccctgaccccagtctgatccagaatcactggagcatatttctctagtctggtaagcatcagaatgtgctagctcaggaattgaggatccctctttacttctcagacactgtatcactgccttcaaggtaccacattcctctttcagtaactgaacggcaacatagtgttccctctttaaggtttcagtttctgaaatatgtctggattccatgtccaaaatttcagcagcatgtagttcttgcatcttctcaattttttcagtaaactgactgattatttcagtaacttcttctgaggaacattcactctgtaaattaatttgtattcctgcatttttaacaagaatttgtggagtctgattgctgctactgatcttcagagtcccatctgtctgggatgcaatgctcttactcagttttataggaagtggctcaaacatgcaggcctttttgctttcttgtacctcagtctcatcttctttttctaaaatggacaatttctcttttgcctctgcgaggtgatccctaacttggcttaagtctttctgaagagatgtcatatttgtttcttttaccaaaagctcttcttgaagtttttcagccttttctttataactggcaagttctgctttggtagccactgattcagctctaagagcctcgagttcattaaaaaatccactttcttcattgctatgaaatagctcagtagttgtcttgagaacttcaacatcttgagggcttcttttcttttctttctctctctgttttttctcattgccctccaatagcttctgtagttctagcagcttcttttctttttctaaaacatttttttctgcaatttctacttgttctttttctaaaatcaaactagtatgcatttcaacaacctggctttctaattctgatattctcaaggttaatgctgatatatctgaccccaactcatcttctcttagttgatttaaattctgaatatttgttctttcaggttctgatgaaattgtttgattatcttgacagaattttgcatattcctgaactgcctcaagttggatttgactgacaagagcagcagccactttttcttcaactattttctgtaggtttacaatcttcttttgaagcatttctgtttcaaactggccttgttcttgcatgtcttttatttgtttataacactgggtaagttctaagtcctttgcactaacagtgctctcaagttgtagcaaccttgtttccaaattaattatggaacctttgccattttcttcaaaagatttgaagtatgtctgattttctagggatttaagagcatcctctgtaaggactacttctagttcaggtttgtctttgctcagatgatctatagccacgttaacactattctctggtatgctttgaatcttttccacactttcacgttctctctttaagctgaataattcctgtgttagctgattcattttaaaattggtttctttaagtacatttttcatgaaggtcatttcttcattagcggtttctacttgctgttccaaggccagcttttcagctataaccacatccaattgatgttttaaactgtctgcttcttctgagagggaatgagcattcattgatgtcttctgtccaatatttgccaattcctgttgaagtttttcaatcacttcattgagctgctctatttcttcttctctatttctcttcacacattcttgatcactcatcaaacattctatttgggtttcaagatcccttatcagttcatttttttcttcaataaccttgttatctgttgtaattttaagttgctgctggagtttcgtaacttgttcatttaattggtcaatttctacctctttttcctgtattatttgagcaaatttcccaaatagcacatgttggtcttgagtagacatggcatcagattcctttatggcaagtcccagtttctccatgtcatccttaaataatttgttttcctgttcaagttcttgtaggcgggtagtagattcctttttctgtatttctaattgcatatgtaattgttgaacttcttcattcttattttccagttcttctctaaactgttctaattgctcttctaagtttgtaatctctttttcctttctgtctatggcatctcgttcagcctgcaattgtacttctagggacaattctggtttagcttctacagctccaaagtgttttcggtcctctaccttttgaaaagtatctgcactcacaagaagcgcctgctccagttctcttactctgaactccagtttctctatttcttcattcctttcttgtatatccctttgaagctgctctttagagagcaaaagctcactgcatttgtctgttttttctttcagatgatttgctaactgttcaacctctctagtttgatgttcactgataggctggaatcgaggaacaaccttaagttgctgttctagtttctgtatttcctgttggaatacatctctctcatgttctctgtcaatggcttgctcatctaaaaattttctcattttttctaactgcttttccaatgcttggttttgctgtcttaaatccattagttcagtatttttttcttgttccagctctataaacctactgacttgttcttccacatctatttctagagctttcacttgtttttgaaggtcatcacgtactttttcagcttgacattgtacttctagtttttccttcattaatttttctgtctcctgtagtaattctgctcctggtgctgcatcgactgcagcatctactagtcgttgttcaactgggcctgcctctgctttcatagcttccttttgtctggacagtaattctctttcttcttggatctgctgttgctctgcctccaattcttgcaacctgttacttgcacataacaactcctgctcaagacgatctattatatcagttttttcctgaatttgcctttcaaaaagagttttttcatctgcatagccatcaatgacgccctcagccttactgagctccacagctagctgttctctggccctggactcctcatgaaggcgctctcgaagttcctcttggcacttaagggactctgttgcttcttgtttctgtctaaatgactcacgcatcaactctgtctgtgtcactttcgcatgttcaagctgactgctagtttcacttatggcttctaggagtttttcaactgctgcttgtagtcgagagctaatgttcagcataagttcttcattttcagggtctatttcagttccagcaaaaccactcctcacaagtcgttgtgacagctctgttccttcctcagttacttttgaccacatgttaatgtcatttcttggcatatcacttccagaataagagggaatggattcatctgtaactcttgtatgttcctcatggacacatgactttacagatgcctctgcttctgacctccaaattaggctggcagatgactggcttttactagatctatctagaatcccaaggacatggcgaccaattgtttcttcaacagctgctgttgtctttacaacttctaagaggatcttcaaaagtctattattagctttctggagtgcatacactgtctttcttgtttgagttccatactgactgcgttccatactgatgatccaatggggaagccaaaatcttaggggccaaattcctccatgcaagctttcattagacaaaatctcaggaggcacatcttcaggttttctgtctaattccttttctttaaatgtttgttcttcaacttctccttggttttcatttccattctgtgtttgcgtactgctgttgcgcagctcacaacacagcttctctcttccagctaaagacagctgctttagtgcttccagctcctctaaaagcaccctctctctctctgaaaccaggttttcattatctatggaggatctctgggctaattgtctattaagtctcttaatctcttcttgtagctgttcctggtcttctcgctgtctctccatttgccgcatatgtgcttgccttaacaattccgttgcctgttgatgttcttggtattgtcgtacaagttcctgtctcatatcttccaactgttcttcattcaacattagttgtctagaagcatccatgcttgacactgaaatctcatcatgaatagactgtctaactataaatgttttatctttggagaacatttcttctgaaatagtcagcacacagtcctttgattctggtatatcatggggatcactatttgataataaaatttcctttccatgttctcctaactctttactaagtggtttaaattcttctttaaatttcacatccactgtctcaaaagtctgaaaaccaatttgatcctgtgataatttcatttcattaaaataatgttgttcttgctgacacacagcatgtgcttgctttgatgatgcagtattttcttttcccccagatattctagacagttcagtttgttgagcaaatgctatactcattgacacaataaccttagctacttcttcttctaattgttcttggtattgtttttcaagcaacttaacgatatttgtttcctctttcactccaaattcaccagaaaactctattgtaccatcaatattctttttcacacaacttccagggtacattgttctctgtgcatcagattctgtaattaccaccgaatcaacaggtaagcttggcggaaccgtggactcactaacagcttgaagcctcttctgtaaacagtggatctctgcctcatagttttgttcagtttctttcaactgttgctgcaaagaggatatgaggctttctaattcttgaacttgttcttcaagtttagttttttcaagatcttgcagagaagataacttgcttttatgattgacatcaatgtcttccaaattggtcatctgagaatggattgataaaaactctgtttcctcttttggaaggttttcttctccaaattcaagtttcataccatctgtctgctgtccccagatcttgcttagtcgtgtttgaagtaccaagagtttgttgtattcttctgttactttgttgagaagagtgtgcatattttcttgaaagtcttgaacttcatatctataatcttgtaattctggatcttcattttcagaaatgtaatcaccagaattctctttgtcttctgcatttacttcacattttaaagcaggagtataatattcaccaaggacactgcataaagtctgtaaaaaataagaacattcttcagacactgccttttgaagttttccaatgagcagatgtaaaggctttccttcatcacctgtttcttgtgttttcatagtctgtagttctaactggtgtattttctgaagttccttgatcttttcctcttgagcaaaaataagctcttctttaagactgcaaagagctttatctttttcattttccatatattcacgaacctgatccacatgagttgaataaaccagagagaggcaaatgcgttgggcttccatctgtagccttaaatcattctgttctgatttaagtacattgagttctttctgaagtttatcattttcacttggttgagttgctctaagtgatgattcctttgttacagatggtaagtgatccaaaatcaactgttcttgcttactttcttctccaacagtcatattttcaaaagaaactttatcttccaccattatttttgattcttcaccaaaacttttatttactttagaaactgatccttcagcacccctgcttgtcatggtcacaactccatctaataaagagcttacttgagtatcacatgactgtacattttctgccctgttgtggttaataatgatttctagctctctacatctcaatgaaacttgttctttctcttgctttaaagatttaacttcttcatttagaaaactaatctcaccatgtttctgtttcaattgttcagaaagatcagacagtctctgtgacagctctaatttctctcgcttggttacctcaagtttttccatgagttctgttgtatccttttcaacaacctcacccatttccaatgtttctgctacaaaagttttgtcttcatcaaagacagaacttttcattttcactgtagttggatttattctttgcaaatgaagctcttcattaagtgctttaagtttacttttatactctaattcctgtttatttttactgtcttctaaatcatcttttactttgagaaggcaagcatactcctcttgtaactcttgatagttaacttcaaagtttttttcagcaaatgaaaaagtgttcctttgcttttcaatctcttcatttagctgaatacattgttgtttgaggtcctcattttcctctataagtatttctatttctttttcccacacagagtctttggatttggacttaatggagtctaagaaaatcaatctttcttcttggctaacaggagtatgtattttcaacatgtcttcaagggttttcttttcatctttaagaatgctattctctgcttcaagttgtgcaaatttttcttgaagatcattctctttttccttcatctgtttttctaacaattctgttttaagttgtaattcttgaacttcttgttcaagtgtacccttttctttttcttcttgtctgagtatttcaatttctttttgaagttcattgatttgaagagtcatttcttctgactttgaatttacaagagactgctgtaaatcttttagctttgaaatttccaaaattaattgattctgcttagttatcaaattgtccttttcaaactgcatggtttctatcttttgactcatttcattctgtaaaccatctatctgctgtttatagtgaatgcctaaattatctttaagtttttcaatatttattcgatgttcaatttctaaatcttccttcagtttggaaagctcttcttcgtgactaaatagaagctgtgttctcagcctctctaattcagcttcttgtgattcagccattctgtctaacacagcattcttttctttttctaacatttcaagttttatcttgtaatttgtaacttctgcttcatgttttaattctagttcctttctggattcagatgcagaaacaatctcagctttcaaatcttccactgtactaagggacttatgtgcttcattaagtttactttcttgttcagctattgtctgtctagctctctgaatctgttcccttgaaaagctcaattcttcaacaaggtcttcaagctgtctctgtagagcacacttttcttctaaaattagtcctagttcttccttgagtttttccttttgagagttagtatcttgcaattttatattcagttcatttattgccacattcattaactttatctgatcttcattaactgtaatatttgaatatgaccttaaagcattctccatttctcccttatgccgtgttttcatttcctccatctgtgccatgtgttgtcttattaattcttgtttcatttgcactatctgctgcccatacatctcatccagctctgcccggagttgttctaactttctttgtgtttcttgttccattcgttgtactatatcagtttcgaactggctgtctttatgatttctcttctgaagttcttcgactgtccccattaactgttttatttcttcagaagactgtctttctttttgcttagaattagtcagctctaatttcatgttttttatttcttggttcttttgcacaatctgttcttgtaattctcctagtaatttatcagcagttgttaatttatcctttagctcaagagttttcttttcttcttctattatttttgtgtttaattcttcaatgattgtctccttttcctgtatttcttctttatttgagttttctacttttttatcttgttccatttcatatactttaattttctcttgcaagaaactaatttgcattgtgaagtcttctttctttttctgataatcttctaataagtggtcttgttcttcaagctgctgttgatgagtgaggatctgttgtttggcttgtagtaagtctgcagctgtgctactatgagtgctgtttctcagagtttcactagcctgtaattgctgaaattgaatctgtaatttttgactctgttctgtcaactctaaaaattctctcattgtctcatccttttctcttcttgcttgttgtaaattagcagtgagctgggttataatgccatctctttgtttaatggcagcttcaaattcttgtaactgctgcagtccttcagtcccataggtaaccctcatttcttccagctctctgtttagctcttcaatctcatgctgcttcccagccaactcactttccatcatctctagatgagtcggactgtcttgtgctccttgttcagaataagaatcatcaacaccaaattcttcttcccttaataaatttgtaggctttcctgttctcatcacaaaactgcaaccatttacctctgaactgcagtcatctgctgtggttgaaatttcactttccagttccacagagaagccctgctcatgactggttatttctccactatgtagagttctcattattgtagattcaggaatcacagttgattctactctctgagaactatttatgtacatttcattacactgtgattgatcaatattcaaatcatggtgtgctgacacatcatgtttactgcttgacgtttttctcttttttttctgcttcttggaaggactctgcccatccgactgagcttttctttgtcgaaactgggcaagcttggctttgccggcctccagcttcttctgtctctcctcgtcctccatggcctctgcaaggaaggcaggggaaaacaggggttgaggggtggttggggatagaaaggaaaggtcgatttggacggaggtgggacggcaagctccacggcctagagagccgattcggtccggcgctcccccgcccgaagtggaagcagtctccgcgctcactggcggatcgtcctcagccgcacgggaagcgccgtcaccgccgccgccgccgccatcttcgtctccacgta

SEQ ID NO: 14143 - RNA, 14476 nt, Homo sapiens
  source 1..14476: mol_type = other RNA
gctgggattacaggcatgagccaccgcacctggccttccctgcttcctctctagaatccaattagggatgtttgttactactcatattgattaaaacagttaacaaacttttttctttttaaaatgtgagatcagtgaactctggttttaagataatctgaaacaaggtccttgggagtaataaaattggtcacattctgtaaagcacattctgtttaggaatcaacttatctcaaattgtaactcggggcctaactatatgagatggctgaaaaaataccacatcgtctgttttcactaggtgatgccaaaatattttgctttatgtatattacagttctttttaaaacactggaagactcatgttaaactctaattgtgaaggcagaatctctgctaatttttcagattaaaattctctttgaaaaaatacagtctgtattcatgaattgtaaaatatgtgcttcagtgagcagagttagggaatccaggaacttgggtggggaaaaattacatctttatttgcactaataatttctaactgcaatttagtatttatttcaattatgaatttgggcagcattttattagcagtatccatgattttgtcaatagaaatctcagatattttcatattacagatgttacagatttcttgaagtatctagttacgaccccgagataaggctagtctaatgtttagtgaatagttttagacttcttaacagatttcatttttaatcacagactaattaattattgagatgcataaacaagtgtgattgcagaggcctactatcataaggaggcgtggtggtcaaacaatggcactgaactcagcttgatcagatcatttgtccatctgtttttttctccactgtctcttagagcagaatagccttgaatggcaagccatgctagctgaaaaaggtttttacccacaacctgccccttcaactaactgctttagagtacgtttgctatttttagaattcctcttattggaacccagcttctaatgtggaaaatttaagtatagttggctccttttatttgtgggttctgtatcctctgattcaaccaactgcaggttcaaaatactaaaaataaaaccccacaataaaaaaatacagtattagcaactatttacataatgttcacattgtattaggtatcaaataatctggagatgatttgaagtacacaggaggatgtatgtagactatctgcaaatagcacattgttttataagagacttaagcattcgcggactgtaatatccaagggggatcctggaactaatcccccacacatgccgagggatgactgaaattagaaatgttcaagcatgtacaactttctaccatgcctgtttgtgttggtataaatcatggaacatcaaataataagacaaaatcctccaggtgtaagcatcaaatactagtcctcttgctgttttagtgagttgccatgttattgaggaggactccagatgagaaataacattgcgatctgtattatctctgtgagagcctcccagtctgaatttggcttggacaacagggatactgtttaattcggctgcaatgtgattaagatcttttgagttaatgatttcttcatctttttagtgggccatggatttgtgagaacacatctttggaaacaagtaacactaactgtaatatagtaaatactgattaatcatgaaataccaatatagcttttaaaaaacactatgtagatgtaaagttgatacaaagacacatggaaaactttcaacagtattaactctaagattaggacaactttctctgaatctctcactcctacatatttgacataagtaatgagatgctatgtaccaagaactatggctcagttaaaaatgaagaaggttcaaatacagtgtggtgaaaatggtgaagtcatttttatttcagtacttgacaaaataccccataaaattcaaaacttctaccattatacaaaaataggtctctacaagtgatattatctgtcttcatcaccagtagaatatattaggcaaaacatgtaacttcagtagccttataagaaaagtgcaggacacctcgagctacacattcagcagtattgtaatgcgtaaaagtttaatcttttcacccatttgataaatacacaaggtttataatttaatgttttaaattagcattccacaaatatacaggtaattcaataattattgtgcatgaatacatacacaatgcttatatatacaaattccagtttgttttcatgtgctggcaagggatttgtatacaatcataagctgtgttcatattggtcccattgaatattcacaatacaaaagcacaaaagaaccattgatttacaaaaggaaatctatttaaaatcacttcaattaatgatgtttcaaaggattatcttctcatgccagcatgaaattgagtagttgaacctgactgtatagttccaagtcgtctttgcagtgcctctagccgagtgatataatctgttagggctctgtcaggatcgtaattctgaagctgagaacatgctaaagaaccaggattgaaatcagctggagtgcctgggtacctattctgaaatggtaaaggggacctaatatagtccagatctgatcttgagcgatacgtagtatgtcttggttctccatataactccagcccaccagaagaatgataaaatgagtcagtcttttctgcaccttgattcagtccaaagccatctctgttaatattgatggaaacagaacctgtgactcgatgccaccgtcgaaccaaaaatttcattctggaaattgcaatggatactctgacggccgaccgaaacctggtgaagccctttgggcgattggtgatcacctctagatccgtgaaagctggctgcccccccatccgggcaagcagggccaaggtggcatcttcacattcctggaacccacccagtaacagcagcaggtatttcttctggtaaatgagagcctttcgaaaactttctgccctcaagtatttaccataaattctctttaaagtgacatgttcagaatcagggctcagagtttgaagtaaagagtcatttcttagttcagctttcagtttgtatacttcagcctctgcccttttcaaagatttctggagagtcaatttttctctgttccatacttctttttcagaggcaatgatggcttcaatgttggcaccaccattcaatgaaaacctggaagaattatctctaccagctcctgtctgtcgataccacctgatctgctcttccagcttcataaccatgttccttaagtcattcttctcttcagtcagttgactgatatgccctgtcagctcagcattttgtctcagtagtctttcagtcaatgagccacaagaagtacttggggacaccaagctgggctcttcaccttgctggccagttaatttctgtagttgtaaaataatttcatcaatattttcctgaacccaaatgaaatcttcatcatctgctgtttcaaactgtagtctctcagaggctttctggggtagaacctgtagttttgaagctacacattgaagcttttgtctgatcatttctaattcatgattacagccggttcctcctccattcatttcaatcaatttagcgtagtttgattcttttgtttctccttctattttctgttgaagaacccaatttctagttctatcactggttaagctccacgtggttggctcattaaggttctgatacagaattcttctactttctcgtttttcttctcgttctagttcttgcttctggaattcctgcatgattccttgtagtcgctgtccttcaaggtctaacttataaacttgttgtcttttctcttccagctggcgctgaagatcttccactttggactggagctcatgcatttttttctgtccctcagtgttggcctcctgttctgtctgcagtgttttcctgtgaacctgcctatctttttccatttgctgtcgtgtttgcaaagaatccagtttatatttttcagtctcatttaacaattctactatgcgactgtgtttttcctctagctgtttctgcagctctttcagtaggtcctctgagggcaagggtggccgagactgtccagtaccatcactgctctgcagctgtgcgtgcaattcccgctccctatctagggtactactcatttcccgaattcgaactttctcagattcaagaagtacctgaagctctaagtttcgaccttgttcttctgacaactgggcatcatatagcattctctgtgattctattttttgctgggattcgttcagtagttgtttctgttgttccaaaagtagatttagctgaagattcctttgtttctgactctcaagtgaaaacttcagatcctcaagttcttctttatcccgttcttcactgcgtcccaacttggctttctctttctccaaagcccactggagctctcttgattttttctgttcacttgctaatgtgtcattaagcaaatgtacttcatctgtcttatctttaacttccaacctgaaagcctccaattcttttaggtgtttatgctgtgccttgagtgttgtttctagttccaatttagtttgtgcaagctcactcttcagttcagcaaccaccattttctcagaactcagctgctcctgcagttccgttgctctgtctttcatactgctgagctccacttgcatctccagcatttgagactgcttctgctgtatattatattccaagagttcttggcttggtttctcactctcttgttctcttttcagagtaattttcctaccattcatttgtgcatgcagtgcctgaatttcagataacaaactccttctatctgctttctggaggcattccatagctgcttgatattcaacaccctgttcttgtattctctgttccaaacagtttagtaaaccaactgcatctgtagtacctagagctgtcagctccgtccgaaatgctgctagtaaaacactacgctcttctaagaaaacttgttgaagggcaagcagtagttcacctcgccagtctgagaagctctcatgagattgagaactatcataaacctcggcttctctttgcagttgcatctttgtaattaaatcctttagagatgagattgtattgatgtaagcttttctctcttctagccaaggttctgaaacctgctgaatagaatggtcctctccatcactatagggagactcagtgagagaaagcacctgcatgccttcattatggacagctctcagtaatccctttattttctttggaaaggaatctgttgcactttcactttcttctcctcggccttctgatgctatgtcaaatccctgactgtgtgtaagataaattccctgaccccagtctgatccagaatcactggagcatatttctctagtctggtaagcatcagaatgtgctagctcaggaattgaggatccctctttacttctcagacactgtatcactgccttcaaggtaccacattcctctttcagtaactgaacggcaacatagtgttccctctttaaggtttcagtttctgaaatatgtctggattccatgtccaaaatttcagcagcatgtagttcttgcatcttctcaattttttcagtaaactgactgattatttcagtaacttcttctgaggaacattcactctgtaaattaatttgtattcctgcatttttaacaagaatttgtggagtctgattgctgctactgatcttcagagtcccatctgtctgggatgcaatgctcttactcagttttataggaagtggctcaaacatgcaggcctttttgctttcttgtacctcagtctcatcttctttttctaaaatggacaatttctcttttgcctctgcgaggtgatccctaacttggcttaagtctttctgaagagatgtcatatttgtttcttttaccaaaagctcttcttgaagtttttcagccttttctttataactggcaagttctgctttggtagccactgattcagctctaagagcctcgagttcattaaaaaatccactttcttcattgctatgaaatagctcagtagttgtcttgagaacttcaacatcttgagggcttcttttcttttctttctctctctgttttttctcattgccctccaatagcttctgtagttctagcagcttcttttctttttctaaaacatttttttctgcaatttctacttgttctttttctaaaatcaaactagtatgcatttcaacaacctggctttctaattctgatattctcaaggttaatgctgatatatctgaccccaactcatcttctcttagttgatttaaattctgaatatttgttctttcaggttctgatgaaattgtttgattatcttgacagaattttgcatattcctgaactgcctcaagttggatttgactgacaagagcagcagccactttttcttcaactattttctgtaggtttacaatcttcttttgaagcatttctgtttcaaactggccttgttcttgcatgtcttttatttgtttataacactgggtaagttctaagtcctttgcactaacagtgctctcaagttgtagcaaccttgtttccaaattaattatggaacctttgccattttcttcaaaagatttgaagtatgtctgattttctagggatttaagagcatcctctgtaaggactacttctagttcaggtttgtctttgctcagatgatctatagccacgttaacactattctctggtatgctttgaatcttttccacactttcacgttctctctttaagctgaataattcctgtgttagctgattcattttaaaattggtttctttaagtacatttttcatgaaggtcatttcttcattagcggtttctacttgctgttccaaggccagcttttcagctataaccacatccaattgatgttttaaactgtctgcttcttctgagagggaatgagcattcattgatgtcttctgtccaatatttgccaattcctgttgaagtttttcaatcacttcattgagctgctctatttcttcttctctatttctcttcacacattcttgatcactcatcaaacattctatttgggtttcaagatcccttatcagttcatttttttcttcaataaccttgttatctgttgtaattttaagttgctgctggagtttcgtaacttgttcatttaattggtcaatttctacctctttttcctgtattatttgagcaaatttcccaaatagcacatgttggtcttgagtagacatggcatcagattcctttatggcaagtcccagtttctccatgtcatccttaaataatttgttttcctgttcaagttcttgtaggcgggtagtagattcctttttctgtatttctaattgcatatgtaattgttgaacttcttcattcttattttccagttcttctctaaactgttctaattgctcttctaagtttgtaatctctttttcctttctgtctatggcatctcgttcagcctgcaattgtacttctagggacaattctggtttagcttctacagctccaaagtgttttcggtcctctaccttttgaaaagtatctgcactcacaagaagcgcctgctccagttctcttactctgaactccagtttctctatttcttcattcctttcttgtatatccctttgaagctgctctttagagagcaaaagctcactgcatttgtctgttttttctttcagatgatttgctaactgttcaacctctctagtttgatgttcactgataggctggaatcgaggaacaaccttaagttgctgttctagtttctgtatttcctgttggaatacatctctctcatgttctctgtcaatggcttgctcatctaaaaattttctcattttttctaactgcttttccaatgcttggttttgctgtcttaaatccattagttcagtatttttttcttgttccagctctataaacctactgacttgttcttccacatctatttctagagctttcacttgtttttgaaggtcatcacgtactttttcagcttgacattgtacttctagtttttccttcattaatttttctgtctcctgtagtaattgttgttcaactgggcctgcctctgctttcatagcttccttttgtctggacagtaattctctttcttcttggatctgctgttgctctgcctccaattcttgcaacctgttacttgcacataacaactcctgctcaagacgatctattatatcagttttttcctgaatttgcctttcaaaaagagttttttcatctgcatagccatcaatgacgccctcagccttactgagctccacagctagctgttctctggccctggactcctcatgaaggcgctctcgaagttcctcttggcacttaagggactctgttgcttcttgtttctgtctaaatgactcacgcatcaactctgtctgtgtcactttcgcatgttcaagctgactgctagtttcacttatggcttctaggagtttttcaactgctgcttgtagtcgagagctaatgttcagcataagttcttcattttcagggtctatttcagttccagcaaaaccactcctcacaagtcgttgtgacagctctgttccttcctcagttacttttgaccacatgttaatgtcatttcttggcatatcacttccagaataagagggaatggattcatctgtaactcttgtatgttcctcatggacacatgactttacagatgcctctgcttctgacctccaaattaggctggcagatgactggcttttactagatctatctagaatcccaaggacatggcgaccaattgtttcttcaacagctgctgttgtctttacaacttctaagaggatcttcaaaagtctattattagctttctggagtgcatacactgtctttcttgtttgagttccatactgactgcgttccatactgatgatccaatggggaagccaaaatcttaggggccaaattcctccatgcaagctttcattagacaaaatctcaggaggcacatcttcaggttttctgtctaattccttttctttaaatgtttgttcttcaacttctccttggttttcatttccattctgtgtttgcgtactgctgttgcgcagctcacaacacagcttctctcttccagctaaagacagctgctttagtgcttccagctcctctaaaagcaccctctctctctctgaaaccaggttttcattatctatggaggatctctgggctaattgtctattaagtctcttaatctcttcttgtagctgttcctggtcttctcgctgtctctccatttgccgcatatgtgcttgccttaacaattccgttgcctgttgatgttcttggtattgtcgtacaagttcctgtctcatatcttccaactgttcttcattcaacattagttgtctagaagcatccatgcttgacactgaaatctcatcatgaatagactgtctaactataaatgttttatctttggagaacatttcttctgaaatagtcagcacacagtcctttgattctggtatatcatggggatcactatttgataataaaatttcctttccatgttctcctaactctttactaagtggtttaaattcttctttaaatttcacatccactgtctcaaaagtctgaaaaccaatttgatcctgtgataatttcatttcattaaaataatgttgttcttgctgacacacagcatgtgcttgctttgatgatgcagtattttcttttcccccagatattctagacagttcagtttgttgagcaaatgctatactcattgacacaataaccttagctacttcttcttctaattgttcttggtattgtttttcaagcaacttaacgatatttgtttcctctttcactccaaattcaccagaaaactctattgtaccatcaatattctttttcacacaacttccagggtacattgttctctgtgcatcagattctgtaattaccaccgaatcaacaggtaagcttggcggaaccgtggactcactaacagcttgaagcctcttctgtaaacagtggatctctgcctcatagttttgttcagtttctttcaactgttgctgcaaagaggatatgaggctttctaattcttgaacttgttcttcaagtttagttttttcaagatcttgcagagaagataacttgcttttatgattgacatcaatgtcttccaaattggtcatctgagaatggattgataaaaactctgtttcctcttttggaaggttttcttctccaaattcaagtttcataccatctgtctgctgtccccagatcttgcttagtcgtgtttgaagtaccaagagtttgttgtattcttctgttactttgttgagaagagtgtgcatattttcttgaaagtcttgaacttcatatctataatcttgtaattctggatcttcattttcagaaatgtaatcaccagaattctctttgtcttctgcatttacttcacattttaaagcaggagtataatattcaccaaggacactgcataaagtctgtaaaaaataagaacattcttcagacactgccttttgaagttttccaatgagcagatgtaaaggctttccttcatcacctgtttcttgtgttttcatagtctgtagttctaactggtgtattttctgaagttccttgatcttttcctcttgagcaaaaataagctcttctttaagactgcaaagagctttatctttttcattttccatatattcacgaacctgatccacatgagttgaataaaccagagagaggcaaatgcgttgggcttccatctgtagccttaaatcattctgttctgatttaagtacattgagttctttctgaagtttatcattttcacttggttgagttgctctaagtgatgattcctttgttacagatggtaagtgatccaaaatcaactgttcttgcttactttcttctccaacagtcatattttcaaaagaaactttatcttccaccattatttttgattcttcaccaaaacttttatttactttagaaactgatccttcagcacccctgcttgtcatggtcacaactccatctaataaagagcttacttgagtatcacatgactgtacattttctgccctgttgtggttaataatgatttctagctctctacatctcaatgaaacttgttctttctcttgctttaaagatttaacttcttcatttagaaaactaatctcaccatgtttctgtttcaattgttcagaaagatcagacagtctctgtgacagctctaatttctctcgcttggttacctcaagtttttccatgagttctgttgtatccttttcaacaacctcacccatttccaatgtttctgctacaaaagttttgtcttcatcaaagacagaacttttcattttcactgtagttggatttattctttgcaaatgaagctcttcattaagtgctttaagtttacttttatactctaattcctgtttatttttactgtcttctaaatcatcttttactttgagaaggcaagcatactcctcttgtaactcttgatagttaacttcaaagtttttttcagcaaatgaaaaagtgttcctttgcttttcaatctcttcatttagctgaatacattgttgtttgaggtcctcattttcctctataagtatttctatttctttttcccacacagagtctttggatttggacttaatggagtctaagaaaatcaatctttcttcttggctaacaggagtatgtattttcaacatgtcttcaagggttttcttttcatctttaagaatgctattctctgcttcaagttgtgcaaatttttcttgaagatcattctctttttccttcatctgtttttctaacaattctgttttaagttgtaattcttgaacttcttgttcaagtgtacccttttctttttcttcttgtctgagtatttcaatttctttttgaagttcattgatttgaagagtcatttcttctgactttgaatttacaagagactgctgtaaatcttttagctttgaaatttccaaaattaattgattctgcttagttatcaaattgtccttttcaaactgcatggtttctatcttttgactcatttcattctgtaaaccatctatctgctgtttatagtgaatgcctaaattatctttaagtttttcaatatttattcgatgttcaatttctaaatcttccttcagtttggaaagctcttcttcgtgactaaatagaagctgtgttctcagcctctctaattcagcttcttgtgattcagccattctgtctaacacagcattcttttctttttctaacatttcaagttttatcttgtaatttgtaacttctgcttcatgttttaattctagttcctttctggattcagatgcagaaacaatctcagctttcaaatcttccactgtactaagggacttatgtgcttcattaagtttactttcttgttcagctattgtctgtctagctctctgaatctgttcccttgaaaagctcaattcttcaacaaggtcttcaagctgtctctgtagagcacacttttcttctaaaattagtcctagttcttccttgagtttttccttttgagagttagtatcttgcaattttatattcagttcatttattgccacattcattaactttatctgatcttcattaactgtaatatttgaatatgaccttaaagcattctccatttctcccttatgccgtgttttcatttcctccatctgtgccatgtgttgtcttattaattcttgtttcatttgcactatctgctgcccatacatctcatccagctctgcccggagttgttctaactttctttgtgtttcttgttccattcgttgtactatatcagtttcgaactggctgtctttatgatttctcttctgaagttcttcgactgtccccattaactgttttatttcttcagaagactgtctttctttttgcttagaattagtcagctctaatttcatgttttttatttcttggttcttttgcacaatctgttcttgtaattctcctagtaatttatcagcagttgttaatttatcctttagctcaagagttttcttttcttcttctattatttttgtgtttaattcttcaatgattgtctccttttcctgtatttcttctttatttgagttttctacttttttatcttgttccatttcatatactttaattttctcttgcaagaaactaatttgcattgtgaagtcttctttctttttctgataatcttctaataagtggtcttgttcttcaagctgctgttgatgagtgaggatctgttgtttggcttgtagtaagtctgcagctgtgctactatgagtgctgtttctcagagtttcactagcctgtaattgctgaaattgaatctgtaatttttgactctgttctgtcaactctaaaaattctctcattgtctcatccttttctcttcttgcttgttgtaaattagcagtgagctgggttataatgccatctctttgtttaatggcagcttcaaattcttgtaactgctgcagtccttcagtcccataggtaaccctcatttcttccagctctctgtttagctcttcaatctcatgctgcttcccagccaactcactttccatcatctctagatgagtcggactgtcttgtgctccttgttcagaataagaatcatcaacaccaaattcttcttcccttaataaatttgtaggctttcctgttctcatcacaaaactgcaaccatttacctctgaactgcagtcatctgctgtggttgaaatttcactttccagttccacagagaagccctgctcatgactggttatttctccactatgtagagttctcattattgtagattcaggaatcacagttgattctactctctgagaactatttatgtacatttcattacactgtgattgatcaatattcaaatcatggtgtgctgacacatcatgtttactgcttgacgtttttctcttttttttctgcttcttggaaggactctgcccatccgactgagcttttctttgtcgaaactgggcaagcttggctttgccggcctccagcttcttctgtctctcctcgtcctccatggcctctgcaaggaaggcaggggaaaacaggggttgaggggtggttggggatagaaaggaaaggtcgatttggacggaggtgggacggcaagctccacggcctagagagccgattcggtccggcgctcccccgcccgaagtggaagcagtctccgcgctcactggcggatcgtcctcagccgcacgggaagcgccgtcaccgccgccgccgccgccatcttcgtctccacgta

SEQ ID NO: 14144 - RNA, 540 nt, Homo sapiens
  source 1..540: mol_type = other RNA
gctgggattacaggcatgagccaccgcacctggcgttctttttcaaacagctctctaacaccaggcaaatcttttgctgctccaaagtacttgtaacctcggtttcctgggacttcttttccttcatgatccagcattttagggccaacttttccataatcaggacctcccagctcctttatccggacctcccagtgtcctttctcccttagcagcttgttaatttcatcattcaggtcacgaattcgaaattcacctaaaccagcattctgaatctgagccacttttttagagatctctccaatgatctgtcgtctccacttctcagctttaggcagttcagtacattctgaggccagaaagggtcttcgttccttcacttttccctcttccagctgagcctggcgaaatcttgctaaggccgtcatggccttttctgcatttcgggccatggtgtcgctaagggcgccgtcctggagccccgcggcccctgtccaagaaactccacaggcccagaagacgccgacgctcacaggaact

SEQ ID NO: 14145 - RNA, 2383 nt, Homo sapiens
  source 1..2383: mol_type = other RNA
gctgggattacaggcatgagccaccgcacctggctagccaactgattcaaactgaagtaggccaggaagatgaatttcacctacaattccaagtcaaagcaaatgtattccagaggcaggggtggggggtggtgttcctctgggggctttttgcctgctttgtgaatacatacaggccatttagaagtttgaatgctgggaagtaagagggctgtgagtctaaaagttgggaacgtgggggagagtgattttatctgcaacaggttcctgggtcctggtgagttctgtacacccttgatgaccaccgattctgggccaggccaaaggcccatctgggcacaggcgatctcaaggtgagtaaagtcaagatgctgcccttcaacgggaggcaggcagccatgccacactgacaaatatacaggtcccaaaggcagcgcagagaggcaagaccacctggttccaggaggcagcgacatcaggaaaacctttccaagggaggtcatctgtgtaggggtttgaagggtgagcacgaatttgccaagctgaaaagggagccaagggcatcctggtggaggagaacagcttgggcaagagtgtgagccgcaagatgggcaggggggctaggcttggaactggaggagcagagagaatgaggtcagcaggggtcagtcacagaaggttttgggtcctggccaaggagcgatgggagctgcaggaggaatgtggcccaggaggagatgaggctccctctgtgtaaagacggatcacgccatctaccaagtggactataagacacaataggaatgggaaacctgactggccttcacaaaggatcaggggcccagagggagcaccaaggaaggttcctctcagaggtcagctttgggggaaggtggaaaatgcttttgagggcttcagctgctgcaaacctcaacaaatcatattttgccttcaaaggttggccaaagaccactaactattggaaaaacaagagtccactaatagtcatcatcccctccctgtgtatttctttaccattctcaaaatgccaccatctcattgaacctccatatcatcccattttgcagatagggaaactgaggccctgtgatgtcacacaggggtcagcagcagttccagactagaagctacggagcacaaacatctcagccttgggtgtcaggctcaaaacccagctccttgtccgggaggaggtccccggctccatctggcagcccatagtacaggtcttcctcttccttctcaggttcctccccacctgtgtccgaagcctccttctcctccacctttgtccttgggtaccgctgccagttgttgggcagggctatttcccactgctgcccctcttggggctcatcctccaacgttggggcatcaatcagggcaaagtcttggaagcggtccagcgggcacctgcagccctgaggttcctgttgtggggaacaagcttcctccctgtcatgtggagatgcattggggctgctgccttcactggagtccatgtccaggtcatcttggaaggaagccaagggggcagggccctggggacaggccagggggccgggccagctctgagttaggcgtctttccccttcactctcgtctgagcccttgtggatgaccacggcagcctccatccaggcctgaacgtcgccagggccaccttctcctccatcactggttcccagcttcggctgccccatctcaggggccagcaaggagcggtggtcctcactgtagctcatgactttcatctggatgtggctgaagtcaggcaggctctggtcataggcggcttcctcccacagccttacatagggcggctggggactggggctcttcatctcggcagcaagcccattctccagcaggcccatggcctttggggagaggatgccttgaaagtcagagtcagcagggacgaaggtgatcttggggtagcactggcacatgctccagatgatgcccccgatcaccatgacgctgcccatggcatagaaggtgccgtagacctggggccgatcatggctcatgaggaacgtaccgagggccagcaggaaaagccccagcacaatgaagccgatccggaaggtcttctcgtcagccatggctgcctggccagtccctggcctgcacacccccgggagagggggtggctgtagttcagcctaaacaccgagacaggcttacacagggagagaagacactgaaatcgctgcaactcaaggcttcaagggagagcaagatccctttcaatcccgctccagtccctgggcccaccagttcaacagggctggaggcggctcgcttcaacggacccacacccagccacctttactccttgccctctcaccttccctct

SEQ ID NO: 14146 - RNA, 4370 nt, Homo sapiens
  source 1..4370: mol_type = other RNA
gctgggattacaggcatgagccaccgcacctggctatatataccagattcttgagcagataattaaacctcctccaccacaaaacttgaaaataaggtacaagaaggcatgacatgagaatccacctgccccttttcccatctgactgtgatgctgaggtgtggtggaattagccaaaagatgtaggaagaaaacttgggtgagctacacccagaataattaatacttaagtcatcaagggttgattgtacttgcaggagaacgggtaactttcccacataaagctgaaatgctagtacagagaaatagccttccatttgctattacaggatcaatgtgcaggtttgatcactttttttttgaagcattttcttttgccaagaataaaaatcatgtatagctattgcactaccaataggtcaattcatgctacaaatgtccatgtgtttctaggatgccagtggctactgctaccagaaataactccagtcactcccttgactagtgttgctagtttggtctttagggtttacctaagtgagagcatcaatgatgggttaaagtcacagaccacaatgaataaatcacagtctgtgcacacttttggccaggaagagtggcagtggaatcttgcatgtcatttggttgaaattaagactaaatctctatatgtgcacacacccacactcacacccacacgcacacatatcacagggttatagcagaatgaaaacggtgggtaggaatcaccagttgaaggctgtaggtttaaatgatcaggattggcacactcagatcagcccaccagtggtcttcactttgtgaaatggaactaatgccacaaggaaactgcatggttacttcatctgtttacacatctgcttatatgttcagctgaactgtcactgaaaacaggagcaccattcttgggacatgaaacaaggaggaggggaaacattcagataatcaacagttaatagaacaagtaaaaaaataagccaacagcaggtgcggcatctctggtatgcaaaacaactaatgaaagtgttcaaaggaattatcaaggcaggccattaagactataaaccatcaaaagagcagcagcaatagcaagagagaaagaagagggttagcaagagactagatcttcctgaaaaagtggccttggctctacaattgtctaccttgtgctgtccttagaagaacaggcccagtgctacagaataaaaatctccatgccaagccactgccttcagaatggtgatgatgtcttcttacaaaggtaaacccaagatgacaaccacaagcaaaaaaatcacccttttgttttaccatcaacagatgaaatagtccatacagtgccattcaatttcccacaggcagaaaccaaagacctcagaatgagaaagtcatggttttcacgtcacaaatgttacgtgtggtcagattatggagcaatgaaaacatttttctgcgccgctcattacactaaatcttgatgtttctgaagtctcttggagtttgagatgtattggaatagtttttcgcaccaagattaacatggcacagtaggaacaggctactgacaaatccatgtccacttaccttacccacaaggttccctaagggttcccttcattctcacaatatttcattttgagatgacttaaggtcaggtagaagggaccacataggccactcttcatcacttctcctcctagctcagaggctcacaattgaggcacttggcccttttgcactactaacatctggggctggaaacctgttgctggataaatacagctcagcaaatccccaaccatatttctattcactaaggtgttattggattgctcctgtttgtgcatgtctgcacacacatgcacaatttcttgtcctctccctccacacttacagacatacacctggtcatgtggaccatcgaaacacaacttgtttggatggaagaagaaaactctgcagatgctgttatttttagaagcctgcttatccctcctgaatgccaacaattttggcttggcatccatttcaaatcaagcaaggtgcatatccaggacaaagcaatgtgcattatgtctgaagggatccacatcttcagtgaaactcagaatgtggccagaactagctaactacctgaactgaaagcaccccatgttcagattcagaccaactcaaaacacatgtaaggggtgcctattgtatgcagggtaaggtgtcaagtccctttttatttggattaagctcaaataagaaaggacctgaagcgaacgtgggatgtgtatgtgtgtacatgtacacgtttgcaaacacacaggtttatgtgggtattaatatcgagtggaaaatctggctttttatttgtctgtgtctttttttttttttttcagtctgattcgagtatatctgttttggcaagttgtgggcagctctcttttacttttgtcacccagaggcttccgtagacaaaaggaaaggagagaggtgtgttcaaagacccccatggcgaagagcccatcccccaagcctgacacaaccctccctcccagcggacccctcttctggactggcttcgctgttggctacttcagtgcatctgacccccaccccccgcgtgaagacctgagattgagcgtggatttctgttctccaccaactctgcagcaagggccctgccagaggcgtcgcttcctgtcatctcctcttcccgctcccaagtagaggcacctaaacagagattagatttctggtttcaaggcatgtcggaccaagcacgctgaatgaacatgagttagttaattagctcggtctctcttctttccgttccctggtctgaatgtttcttgatggcaaagcgaccaggagagagttgatttgcatcttaagacctatgggtaatgcttctggagtggggagatttatttagcaactgcttgaacttgtgtacggggtcgggaaggaggtggagctgaccccaatggggctatcggagattggggtgtgggtggtgcccactgccacgctgacaccccgggcctcgatgatggcagacaggagctgctgctgctgctggcgcagggtgtcggcgatgagcagcggcagggagttgaagctggcggtgagatgctccagcttcgactccaggctgccaatctgcttctccaggtcttcgctccggtcattgagttctgtgattaagtcatacatgacattctgcatcttggaaaggtccaccagagtgttggcttggtcactcagcttcctctgttccatcttgacgctcctcaactggtggatagcttggaggaacttcctctggtgtttcctcactttggcatggtcaatcttctttagcagctttgtgtgtttatagattaaccatgtttcccgaaggacattggctgcagcattcttgatccgcttggtgagctgagtgtccatcatgaagttatgaacgtgcttctccgctttggtgagttccagctttcgggccaccacggccaccacaagggcagtgcagcctgcacccatgatgccagtgaggagacagacacctttcccacagtatgtgtggggcaccatgtccccataaccaatggaaaggaatgtgatggagatgagccacatggcacccagaaagttactagttacgtcctgctggtcatggtaccaagcaggaagtgatgagccagaaggctgggctggtgattcaggactttcacagacacggacggtccaggcagcaatgatccacagagagatgctgaacacgagcagcacagtgccagggcagatggtcatgagcgtcttcatgacaaagcgggtgttgaagttgatcttgttgagggccccgatgctgcgggacgaggcatcggtgaagagcttgctgtgcagcagcatgactcgggcgatcaggtacaggcgcaggaacatggggatagacaggatgatgtccacatcggcctccgcccgggagggtgtgtaggagaaggccaggcgtgccgtccagaagaacttgtactcgccaggaatggggtggatggcgcacaccagcatctccaggctgatgtacaggatgcgctcgtaggtcatggctatccgccagtcatccgcgccattgtcgatcacgaagagctggacttcacgtgtgtggtaggcgatgatcaagcccaaaaggatgatggtggacagactgataaggcatttcagggccaacgaaaacatggagtccttcctccatctccactccctctgggagggaaaccccctcctccgtcttggggctggactgagaggctggagcagtggggccagctccccgctaaagccagtgcctgctgttctccatccgg

SEQ ID NO: 14147 - RNA, 5498 nt, Homo sapiens
  source 1..5498: mol_type = other RNA
gctgggattacaggcatgagccaccgcacctggctatatataccagattcttgagcagataattaaacctcctccaccacaaaacttgaaaataaggtacaagaaggcatgacatgagaatccacctgccccttttcccatctgactgtgatgctgaggtgtggtggaattagccaaaagatgtaggaagaaaacttgggtgagctacacccagaataattaatacttaagtcatcaagggttgattgtacttgcaggagaacgggtaactttcccacataaagctgaaatgctagtacagagaaatagccttccatttgctattacaggatcaatgtgcaggtttgatcactttttttttgaagcattttcttttgccaagaataaaaatcatgtatagctattgcactaccaataggtcaattcatgctacaaatgtccatgtgtttctaggatgccagtggctactgctaccagaaataactccagtcactcccttgactagtgttgctagtttggtctttagggtttacctaagtgagagcatcaatgatgggttaaagtcacagaccacaatgaataaatcacagtctgtgcacacttttggccaggaagagtggcagtggaatcttgcatgtcatttggttgaaattaagactaaatctctatatgtgcacacacccacactcacacccacacgcacacatatcacagggttatagcagaatgaaaacggtgggtaggaatcaccagttgaaggctgtaggtttaaatgatcaggattggcacactcagatcagcccaccagtggtcttcactttgtgaaatggaactaatgccacaaggaaactgcatggttacttcatctgtttacacatctgcttatatgttcagctgaactgtcactgaaaacaggagcaccattcttgggacatgaaacaaggaggaggggaaacattcagataatcaacagttaatagaacaagtaaaaaaataagccaacagcaggtgcggcatctctggtatgcaaaacaactaatgaaagtgttcaaaggaattatcaaggcaggccattaagactataaaccatcaaaagagcagcagcaatagcaagagagaaagaagagggttagcaagagactagatcttcctgaaaaagtggccttggctctacaattgtctaccttgtgctgtccttagaagaacaggcccagtgctacagaataaaaatctccatgccaagccactgccttcagaatggtgatgatgtcttcttacaaaggtaaacccaagatgacaaccacaagcaaaaaaatcacccttttgttttaccatcaacagatgaaatagtccatacagtgccattcaatttcccacaggcagaaaccaaagacctcagaatgagaaagtcatggttttcacgtcacaaatgttacgtgtggtcagattatggagcaatgaaaacatttttctgcgccgctcattacactaaatcttgatgtttctgaagtctcttggagtttgagatgtattggaatagtttttcgcaccaagattaacatggcacagtaggaacaggctactgacaaatccatgtccacttaccttacccacaaggttccctaagggttcccttcattctcacaatatttcattttgagatgacttaaggtcaggtagaagggaccacataggccactcttcatcacttctcctcctagctcagaggctcacaattgaggcacttggcccttttgcactactaacatctggggctggaaacctgttgctggataaatacagctcagcaaatccccaaccatatttctattcactaaggtgttattggattgctcctgtttgtgcatgtctgcacacacatgcacaatttcttgtcctctccctccacacttacagacatacacctggtcatgtggaccatcgaaacacaacttgtttggatggaagaagaaaactctgcagatgctgttatttttagaagcctgcttatccctcctgaatgccaacaattttggcttggcatccatttcaaatcaagcaaggtgcatatccaggacaaagcaatgtgcattatgtctgaagggatccacatcttcagtgaaactcagaatgtggccagaactagctaactacctgaactgaaagcaccccatgttcagattcagaccaactcaaaacacatgtaaggggtgcctattgtatgcagggtaaggtgtcaagtccctttttatttggattaagctcaaataagaaaggacctgaagcgaacgtgggatgtgtatgtgtgtacatgtacacgtttgcaaacacacaggtttatgtgggtattaatatcgagtggaaaatctggctttttatttgtctgtgtctttttttttttttttcagtctgattcgagtatatctgttttggcaagttgtgggcagctctcttttacttttgtcacccagaggcttccgtagacaaaaggaaaggagagaggtgtgttcaaagacccccatggcgaagagcccatcccccaagcctgacacaaccctccctcccagcggacccctcttctggactggcttcgctgttggctacttcagtgcatctgacccccaccccccgcgtgaagacctgagattgagcgtggatttctgttctccaccaactctgcagcaagggccctgccagaggcgtcgcttcctgtcatctcctcttcccgctcccaagtagaggcacctaaacagagattagatttctggtttcaaggcatgtcggaccaagcacgctgaatgaacatgagttagttaattagctcggtctctcttctttccgttccctggtctgaatgtttcttgatggcaaagcgaccaggagagagttgatttgcatcttaagacctatgggtaatgcttctggagtggggagatttatttagcaactgcttgaacttgtgtacggggtcgggaaggaggtggagctgaccccaatggggctatcggagattggggtgtgggtggtgcccactgccacgctgacaccccgggcctcgatgatggcagacaggagctgctgctgctgctggcgcagggtgtcggcgatgagcagcggcagggagttgaagctggcggtgagatgctccagcttcgactccaggctgccaatctgcttctccaggtcttcgctccggtcattgagttctgtgattaagtcatacatgacattctgcatcttggaaaggtccaccagagtgttggcttggtcactcagcttcctctgttccatcttgacgctcctcaactggtggatagcttggaggaacttcctctggtgtttcctcactttggcatggtcaatcttctttagcagctttgtgtgtttatagattaaccatgtttcccgaaggacattggctgcagcattcttgatccgcttggtgagctgagtgtccatcatgaagttatgaacgtgcttctccgctttggtgagttccagctttcgggccaccacggccaccacaagggcagtgcagcctgcacccatgatgccagtgaggagacagacacctttcccacagtatgtgtggggcaccatgtccccataaccaatggaaaggaatgtgatggagatgagccacatggcacccagaaagttactagttacgtcctgctggtcatggtaccaagcaggaagtgatgagccagaaggctgggctggtgattcaggactttcacagacacggacggtccaggcagcaatgatccacagagagatgctgaacacgagcagcacagtgccagggcagatggtcatgagcgtcttcatgacaaagcgggtgttgaagttgatcttgttgagggccccgatgctgcgggacgaggcatcggtgaagagcttgctgtgcagcagcatgactcgggcgatcaggtacaggcgcaggaacatggggatagacaggatgatgtccacatcggcctccgcccgggagggtgtgtaggagaaggccaggcgtgccgtccagaagaacttgtactcgccaggaatggggtggatggcgcacaccagcatctccaggctgatgtacaggatgcgctcgtaggtcatggctatccgccagtcatccgcgccattgtcgatcacgaagagctggacttcacgtgtgtggtaggcgatgatcaagcccaaaaggatgatggtggacagactgataaggcatttcagggccaacgaaaacatggagtcctttgagtacaaaccccaagagagctcggtctctatcaccataacaacaattccaaacatcccaaaaatcagagcatagtcactcagtcgctttctcttttcaaacagggccctcctgtgtcccagcttatagccaatgttttggtttttccgcttgttggctttggggaaggtggtgctgctggcggtggtgccggcatgctggtggttgtgggtggcattagggtgatggagcagggtctggtgggcatggttgtcctcccgggaggagatgacgatctccggggggttgctagggctgaaaagctggaggggttggccctcagtctcggcctcgatgaggttcctccgggaggcgctgaggcggctgaggggcttcatgaccccaccgctatacttgcaggagctcatggcgatctccgtgaaggggttgctgtcccgccggtgcaccagggggctggcctgtcggtgccggctgcctccgccaggcccacttgtagctgtggaacttggagagtggccaagcaagtggtcattgagattgagctggctgccttgcctggaggaagggtggaggatggcggtggagttggacgaagggggggccctgaaagcggtgggagaggagtgcagcaggccagggtggacgggctggctctggagttgggcgagctgagacaggggatgcggtggctgctgctgctgctgctgctgctgctgctgctgctgctgctgaagctgcggaggctgaggctgcagcgagggtcccaggggctgctggggggctgctggtggcgctggcggtggtggctgctgctgctgttgctgctgctgctgctgctgctgctcatccccagaggatggacaggggcacttggggtcttcatccaagtcccccacccccgagtcatggaagtgcccagaagtgtccatcttggggcctggctgtattccctgcagcacaagcccccaccccaaagccaccctcgctccaaagatgtcctcaaagaaagccaggcatccaatctcccccaccagtatcttggctccagtcctctctttggcttgcttcggttctctggggctgcctggagtccagacgctgccactcaagaatgcattgtattgggcagggagggagagcaggaggggagcttggagaaagaagagggggtgaaagaactctctcaggaggtggtcctctaggagcgtgtgaggccaggctcagcttcactcctcgctggctcaat

SEQ ID NO: 14148 - RNA, 4325 nt, Homo sapiens
  source 1..4325: mol_type = other RNA
gctgggattacaggcatgagccaccgcacctggctatatataccagattcttgagcagataattaaacctcctccaccacaaaacttgaaaataaggtacaagaaggcatgacatgagaatccacctgccccttttcccatctgactgtgatgctgaggtgtggtggaattagccaaaagatgtaggaagaaaacttgggtgagctacacccagaataattaatacttaagtcatcaagggttgattgtacttgcaggagaacgggtaactttcccacataaagctgaaatgctagtacagagaaatagccttccatttgctattacaggatcaatgtgcaggtttgatcactttttttttgaagcattttcttttgccaagaataaaaatcatgtatagctattgcactaccaataggtcaattcatgctacaaatgtccatgtgtttctaggatgccagtggctactgctaccagaaataactccagtcactcccttgactagtgttgctagtttggtctttagggtttacctaagtgagagcatcaatgatgggttaaagtcacagaccacaatgaataaatcacagtctgtgcacacttttggccaggaagagtggcagtggaatcttgcatgtcatttggttgaaattaagactaaatctctatatgtgcacacacccacactcacacccacacgcacacatatcacagggttatagcagaatgaaaacggtgggtaggaatcaccagttgaaggctgtaggtttaaatgatcaggattggcacactcagatcagcccaccagtggtcttcactttgtgaaatggaactaatgccacaaggaaactgcatggttacttcatctgtttacacatctgcttatatgttcagctgaactgtcactgaaaacaggagcaccattcttgggacatgaaacaaggaggaggggaaacattcagataatcaacagttaatagaacaagtaaaaaaataagccaacagcaggtgcggcatctctggtatgcaaaacaactaatgaaagtgttcaaaggaattatcaaggcaggccattaagactataaaccatcaaaagagcagcagcaatagcaagagagaaagaagagggttagcaagagactagatcttcctgaaaaagtggccttggctctacaattgtctaccttgtgctgtccttagaagaacaggcccagtgctacagaataaaaatctccatgccaagccactgccttcagaatggtgatgatgtcttcttacaaaggtaaacccaagatgacaaccacaagcaaaaaaatcacccttttgttttaccatcaacagatgaaatagtccatacagtgccattcaatttcccacaggcagaaaccaaagacctcagaatgagaaagtcatggttttcacgtcacaaatgttacgtgtggtcagattatggagcaatgaaaacatttttctgcgccgctcattacactaaatcttgatgtttctgaagtctcttggagtttgagatgtattggaatagtttttcgcaccaagattaacatggcacagtaggaacaggctactgacaaatccatgtccacttaccttacccacaaggttccctaagggttcccttcattctcacaatatttcattttgagatgacttaaggtcaggtagaagggaccacataggccactcttcatcacttctcctcctagctcagaggctcacaattgaggcacttggcccttttgcactactaacatctggggctggaaacctgttgctggataaatacagctcagcaaatccccaaccatatttctattcactaaggtgttattggattgctcctgtttgtgcatgtctgcacacacatgcacaatttcttgtcctctccctccacacttacagacatacacctggtcatgtggaccatcgaaacacaacttgtttggatggaagaagaaaactctgcagatgctgttatttttagaagcctgcttatccctcctgaatgccaacaattttggcttggcatccatttcaaatcaagcaaggtgcatatccaggacaaagcaatgtgcattatgtctgaagggatccacatcttcagtgaaactcagaatgtggccagaactagctaactacctgaactgaaagcaccccatgttcagattcagaccaactcaaaacacatgtaaggggtgcctattgtatgcagggtaaggtgtcaagtccctttttatttggattaagctcaaataagaaaggacctgaagcgaacgtgggatgtgtatgtgtgtacatgtacacgtttgcaaacacacaggtttatgtgggtattaatatcgagtggaaaatctggctttttatttgtctgtgtctttttttttttttttcagtctgattcgagtatatctgttttggcaagttgtgggcagctctcttttacttttgtcacccagaggcttccgtagacaaaaggaaaggagagaggtgtgttcaaagacccccatggcgaagagcccatcccccaagcctgacacaaccctccctcccagcggacccctcttctggactggcttcgctgttggctacttcagtgcatctgacccccaccccccgcgtgaagacctgagattgagcgtggatttctgttctccaccaactctgcagcaagggccctgccagaggcgtcgcttcctgtcatctcctcttcccgctcccaagtagaggcacctaaacagagattagatttctggtttcaaggcatgtcggaccaagcacgctgaatgaacatgagttagttaattagctcggtctctcttctttccgttccctggtctgaatgtttcttgatggcaaagcgaccaggagagagttgatttgcatcttaagacctatgggtaatgcttctggagtggggagatttatttagcaactgcttgaacttgtgtacggggtcgggaaggaggtggagctgaccccaatggggctatcggagattggggtgtgggtggtgcccactgccacgctgacaccccgggcctcgatgatggcagacaggagctgctgctgctgctggcgcagggtgtcggcgatgagcagcggcagggagttgaagctggcggtgagatgctccagcttcgactccaggctgccaatctgcttctccaggtcttcgctccggtcattgagttctgtgattaagtcatacatgacattctgcatcttggaaaggtccaccagagtgttggcttggtcactcagcttcctctgttccatcttgacgctcctcaactggtggatagcttggaggaacttcctctggtgtttcctcactttggcatggtcaatcttctttagcagctttgtgtgtttatagattaaccatgtttcccgaaggacattggctgcagcattcttgatccgcttggtgagctgagtgtccatcatgaagttatgaacgtgcttctccgctttggtgagttccagctttcgggccaccacggccaccacaagggcagtgcagcctgcacccatgatgccagtgaggagacagacacctttcccacagtatgtgtggggcaccatgtccccataaccaatggaaaggaatgtgatggagatgagccacatggcacccagaaagttactagttacgtcctgctggtcatggtacctttcacagacacggacggtccaggcagcaatgatccacagagagatgctgaacacgagcagcacagtgccagggcagatggtcatgagcgtcttcatgacaaagcgggtgttgaagttgatcttgttgagggccccgatgctgcgggacgaggcatcggtgaagagcttgctgtgcagcagcatgactcgggcgatcaggtacaggcgcaggaacatggggatagacaggatgatgtccacatcggcctccgcccgggagggtgtgtaggagaaggccaggcgtgccgtccagaagaacttgtactcgccaggaatggggtggatggcgcacaccagcatctccaggctgatgtacaggatgcgctcgtaggtcatggctatccgccagtcatccgcgccattgtcgatcacgaagagctggacttcacgtgtgtggtaggcgatgatcaagcccaaaaggatgatggtggacagactgataaggcatttcagggccaacgaaaacatggagtccttcctccatctccactccctctgggagggaaaccccctcctccgtcttggggctggactgagaggctggagcagtggggccagctccccgctaaagccagtgcctgctgttctccatccgg

SEQ ID NO: 14149 - RNA, 4385 nt, Homo sapiens
  source 1..4385: mol_type = other RNA
gctgggattacaggcatgagccaccgcacctggctatatataccagattcttgagcagataattaaacctcctccaccacaaaacttgaaaataaggtacaagaaggcatgacatgagaatccacctgccccttttcccatctgactgtgatgctgaggtgtggtggaattagccaaaagatgtaggaagaaaacttgggtgagctacacccagaataattaatacttaagtcatcaagggttgattgtacttgcaggagaacgggtaactttcccacataaagctgaaatgctagtacagagaaatagccttccatttgctattacaggatcaatgtgcaggtttgatcactttttttttgaagcattttcttttgccaagaataaaaatcatgtatagctattgcactaccaataggtcaattcatgctacaaatgtccatgtgtttctaggatgccagtggctactgctaccagaaataactccagtcactcccttgactagtgttgctagtttggtctttagggtttacctaagtgagagcatcaatgatgggttaaagtcacagaccacaatgaataaatcacagtctgtgcacacttttggccaggaagagtggcagtggaatcttgcatgtcatttggttgaaattaagactaaatctctatatgtgcacacacccacactcacacccacacgcacacatatcacagggttatagcagaatgaaaacggtgggtaggaatcaccagttgaaggctgtaggtttaaatgatcaggattggcacactcagatcagcccaccagtggtcttcactttgtgaaatggaactaatgccacaaggaaactgcatggttacttcatctgtttacacatctgcttatatgttcagctgaactgtcactgaaaacaggagcaccattcttgggacatgaaacaaggaggaggggaaacattcagataatcaacagttaatagaacaagtaaaaaaataagccaacagcaggtgcggcatctctggtatgcaaaacaactaatgaaagtgttcaaaggaattatcaaggcaggccattaagactataaaccatcaaaagagcagcagcaatagcaagagagaaagaagagggttagcaagagactagatcttcctgaaaaagtggccttggctctacaattgtctaccttgtgctgtccttagaagaacaggcccagtgctacagaataaaaatctccatgccaagccactgccttcagaatggtgatgatgtcttcttacaaaggtaaacccaagatgacaaccacaagcaaaaaaatcacccttttgttttaccatcaacagatgaaatagtccatacagtgccattcaatttcccacaggcagaaaccaaagacctcagaatgagaaagtcatggttttcacgtcacaaatgttacgtgtggtcagattatggagcaatgaaaacatttttctgcgccgctcattacactaaatcttgatgtttctgaagtctcttggagtttgagatgtattggaatagtttttcgcaccaagattaacatggcacagtaggaacaggctactgacaaatccatgtccacttaccttacccacaaggttccctaagggttcccttcattctcacaatatttcattttgagatgacttaaggtcaggtagaagggaccacataggccactcttcatcacttctcctcctagctcagaggctcacaattgaggcacttggcccttttgcactactaacatctggggctggaaacctgttgctggataaatacagctcagcaaatccccaaccatatttctattcactaaggtgttattggattgctcctgtttgtgcatgtctgcacacacatgcacaatttcttgtcctctccctccacacttacagacatacacctggtcatgtggaccatcgaaacacaacttgtttggatggaagaagaaaactctgcagatgctgttatttttagaagcctgcttatccctcctgaatgccaacaattttggcttggcatccatttcaaatcaagcaaggtgcatatccaggacaaagcaatgtgcattatgtctgaagggatccacatcttcagtgaaactcagaatgtggccagaactagctaactacctgaactgaaagcaccccatgttcagattcagaccaactcaaaacacatgtaaggggtgcctattgtatgcagggtaaggtgtcaagtccctttttatttggattaagctcaaataagaaaggacctgaagcgaacgtgggatgtgtatgtgtgtacatgtacacgtttgcaaacacacaggtttatgtgggtattaatatcgagtggaaaatctggctttttatttgtctgtgtctttttttttttttttcagtctgattcgagtatatctgttttggcaagttgtgggcagctctcttttacttttgtcacccagaggcttccgtagacaaaaggaaaggagagaggtgtgttcaaagacccccatggcgaagagcccatcccccaagcctgacacaaccctccctcccagcggacccctcttctggactggcttcgctgttggctacttcagtgcatctgacccccaccccccgcgtgaagacctgagattgagcgtggatttctgttctccaccaactctgcagcaagggccctgccagaggcgtcgcttcctgtcatctcctcttcccgctcccaagtagaggcacctaaacagagattagatttctggtttcaaggcatgtcggaccaagcacgctgaatgaacatgagttagttaattagctcggtctctcttctttccgttccctggtctgaatgtttcttgatggcaaagcgaccaggagagagttgatttgcatcttaagacctatgggtaatgcttctggagtggggagatttatttagcaactgcttgaacttgtgtacggggtcgggaaggaggtggagctgaccccaatggggctatcggagattggggtgtgggtggtgcccactgccacgctgacaccccgggcctcgatgatggcagacaggagctgctgctgctgctggcgcagggtgtcggcgatgagcagcggcagggagttgaagctggcggtgagatgctccagcttcgactccaggctgccaatctgcttctccaggtcttcgctccggtcattgagttctgtgattaagtcatacatgacattctgcatcttggaaaggtccaccagagtgttggcttggtcactcagcttcctctgttccatcttgacgctcctcaactggtggatagcttggaggaacttcctctggtgtttcctcactttggcatggtcaatcttctttagcagctttgtgtgtttatagattaaccatgtttcccgaaggacattggctgcagcattcttgatccgcttggtgagctgagtgtccatcatgaagttatgaacgtgcttctccgctttggtgagttccagctttcgggccaccacggccaccacaagggcagtgcagcctgcacccatgatgccagtgaggagacagacacctttcccacagtatgtgtggggcaccatgtccccataaccaatggaaaggaatgtgatggagatgagccacatggcacccagaaagttactagttacgtcctgctggtcatggtacctttcacagacacggacggtccaggcagcaatgatccacagagagatgctgaacacgagcagcacagtgccagggcagatggtcatgagcgtcttcatgacaaagcgggtgttgaagttgatcttgttgagggccccgatgctgcgggacgaggcatcggtgaagagcttgctgtgcagcagcatgactcgggcgatcaggtacaggcgcaggaacatggggatagacaggatgatgtccacatcggcctccgcccgggagggtgtgtaggagaaggccaggcgtgccgtccagaagaacttgtactcgccaggaatggggtggatggcgcacaccagcatctccaggctgatgtacaggatgcgctcgtaggtcatggctatccgccagtcatccgcgccattgtcgatcacgaagagctggacttcacgtgtgtggtaggcgatgatcaagcccaaaaggatgatggtggacagactgataaggcatttcagggccaacgaaaacatggagtcctttataggtctctccatctataacctgaagcaaaacaccaaacaactgtccttgcagatgtcgcgtggcaggcctggtatcagcaagctctaaggagtaggtgccagctcagtccctgcaaggagtgtcctttaagctgactttcctgttaatttgacactgagcagcactcctgtccttt

SEQ ID NO: 14150 - RNA, 5453 nt, Homo sapiens
  source 1..5453: mol_type = other RNA
gctgggattacaggcatgagccaccgcacctggctatatataccagattcttgagcagataattaaacctcctccaccacaaaacttgaaaataaggtacaagaaggcatgacatgagaatccacctgccccttttcccatctgactgtgatgctgaggtgtggtggaattagccaaaagatgtaggaagaaaacttgggtgagctacacccagaataattaatacttaagtcatcaagggttgattgtacttgcaggagaacgggtaactttcccacataaagctgaaatgctagtacagagaaatagccttccatttgctattacaggatcaatgtgcaggtttgatcactttttttttgaagcattttcttttgccaagaataaaaatcatgtatagctattgcactaccaataggtcaattcatgctacaaatgtccatgtgtttctaggatgccagtggctactgctaccagaaataactccagtcactcccttgactagtgttgctagtttggtctttagggtttacctaagtgagagcatcaatgatgggttaaagtcacagaccacaatgaataaatcacagtctgtgcacacttttggccaggaagagtggcagtggaatcttgcatgtcatttggttgaaattaagactaaatctctatatgtgcacacacccacactcacacccacacgcacacatatcacagggttatagcagaatgaaaacggtgggtaggaatcaccagttgaaggctgtaggtttaaatgatcaggattggcacactcagatcagcccaccagtggtcttcactttgtgaaatggaactaatgccacaaggaaactgcatggttacttcatctgtttacacatctgcttatatgttcagctgaactgtcactgaaaacaggagcaccattcttgggacatgaaacaaggaggaggggaaacattcagataatcaacagttaatagaacaagtaaaaaaataagccaacagcaggtgcggcatctctggtatgcaaaacaactaatgaaagtgttcaaaggaattatcaaggcaggccattaagactataaaccatcaaaagagcagcagcaatagcaagagagaaagaagagggttagcaagagactagatcttcctgaaaaagtggccttggctctacaattgtctaccttgtgctgtccttagaagaacaggcccagtgctacagaataaaaatctccatgccaagccactgccttcagaatggtgatgatgtcttcttacaaaggtaaacccaagatgacaaccacaagcaaaaaaatcacccttttgttttaccatcaacagatgaaatagtccatacagtgccattcaatttcccacaggcagaaaccaaagacctcagaatgagaaagtcatggttttcacgtcacaaatgttacgtgtggtcagattatggagcaatgaaaacatttttctgcgccgctcattacactaaatcttgatgtttctgaagtctcttggagtttgagatgtattggaatagtttttcgcaccaagattaacatggcacagtaggaacaggctactgacaaatccatgtccacttaccttacccacaaggttccctaagggttcccttcattctcacaatatttcattttgagatgacttaaggtcaggtagaagggaccacataggccactcttcatcacttctcctcctagctcagaggctcacaattgaggcacttggcccttttgcactactaacatctggggctggaaacctgttgctggataaatacagctcagcaaatccccaaccatatttctattcactaaggtgttattggattgctcctgtttgtgcatgtctgcacacacatgcacaatttcttgtcctctccctccacacttacagacatacacctggtcatgtggaccatcgaaacacaacttgtttggatggaagaagaaaactctgcagatgctgttatttttagaagcctgcttatccctcctgaatgccaacaattttggcttggcatccatttcaaatcaagcaaggtgcatatccaggacaaagcaatgtgcattatgtctgaagggatccacatcttcagtgaaactcagaatgtggccagaactagctaactacctgaactgaaagcaccccatgttcagattcagaccaactcaaaacacatgtaaggggtgcctattgtatgcagggtaaggtgtcaagtccctttttatttggattaagctcaaataagaaaggacctgaagcgaacgtgggatgtgtatgtgtgtacatgtacacgtttgcaaacacacaggtttatgtgggtattaatatcgagtggaaaatctggctttttatttgtctgtgtctttttttttttttttcagtctgattcgagtatatctgttttggcaagttgtgggcagctctcttttacttttgtcacccagaggcttccgtagacaaaaggaaaggagagaggtgtgttcaaagacccccatggcgaagagcccatcccccaagcctgacacaaccctccctcccagcggacccctcttctggactggcttcgctgttggctacttcagtgcatctgacccccaccccccgcgtgaagacctgagattgagcgtggatttctgttctccaccaactctgcagcaagggccctgccagaggcgtcgcttcctgtcatctcctcttcccgctcccaagtagaggcacctaaacagagattagatttctggtttcaaggcatgtcggaccaagcacgctgaatgaacatgagttagttaattagctcggtctctcttctttccgttccctggtctgaatgtttcttgatggcaaagcgaccaggagagagttgatttgcatcttaagacctatgggtaatgcttctggagtggggagatttatttagcaactgcttgaacttgtgtacggggtcgggaaggaggtggagctgaccccaatggggctatcggagattggggtgtgggtggtgcccactgccacgctgacaccccgggcctcgatgatggcagacaggagctgctgctgctgctggcgcagggtgtcggcgatgagcagcggcagggagttgaagctggcggtgagatgctccagcttcgactccaggctgccaatctgcttctccaggtcttcgctccggtcattgagttctgtgattaagtcatacatgacattctgcatcttggaaaggtccaccagagtgttggcttggtcactcagcttcctctgttccatcttgacgctcctcaactggtggatagcttggaggaacttcctctggtgtttcctcactttggcatggtcaatcttctttagcagctttgtgtgtttatagattaaccatgtttcccgaaggacattggctgcagcattcttgatccgcttggtgagctgagtgtccatcatgaagttatgaacgtgcttctccgctttggtgagttccagctttcgggccaccacggccaccacaagggcagtgcagcctgcacccatgatgccagtgaggagacagacacctttcccacagtatgtgtggggcaccatgtccccataaccaatggaaaggaatgtgatggagatgagccacatggcacccagaaagttactagttacgtcctgctggtcatggtacctttcacagacacggacggtccaggcagcaatgatccacagagagatgctgaacacgagcagcacagtgccagggcagatggtcatgagcgtcttcatgacaaagcgggtgttgaagttgatcttgttgagggccccgatgctgcgggacgaggcatcggtgaagagcttgctgtgcagcagcatgactcgggcgatcaggtacaggcgcaggaacatggggatagacaggatgatgtccacatcggcctccgcccgggagggtgtgtaggagaaggccaggcgtgccgtccagaagaacttgtactcgccaggaatggggtggatggcgcacaccagcatctccaggctgatgtacaggatgcgctcgtaggtcatggctatccgccagtcatccgcgccattgtcgatcacgaagagctggacttcacgtgtgtggtaggcgatgatcaagcccaaaaggatgatggtggacagactgataaggcatttcagggccaacgaaaacatggagtcctttgagtacaaaccccaagagagctcggtctctatcaccataacaacaattccaaacatcccaaaaatcagagcatagtcactcagtcgctttctcttttcaaacagggccctcctgtgtcccagcttatagccaatgttttggtttttccgcttgttggctttggggaaggtggtgctgctggcggtggtgccggcatgctggtggttgtgggtggcattagggtgatggagcagggtctggtgggcatggttgtcctcccgggaggagatgacgatctccggggggttgctagggctgaaaagctggaggggttggccctcagtctcggcctcgatgaggttcctccgggaggcgctgaggcggctgaggggcttcatgaccccaccgctatacttgcaggagctcatggcgatctccgtgaaggggttgctgtcccgccggtgcaccagggggctggcctgtcggtgccggctgcctccgccaggcccacttgtagctgtggaacttggagagtggccaagcaagtggtcattgagattgagctggctgccttgcctggaggaagggtggaggatggcggtggagttggacgaagggggggccctgaaagcggtgggagaggagtgcagcaggccagggtggacgggctggctctggagttgggcgagctgagacaggggatgcggtggctgctgctgctgctgctgctgctgctgctgctgctgctgctgaagctgcggaggctgaggctgcagcgagggtcccaggggctgctggggggctgctggtggcgctggcggtggtggctgctgctgctgttgctgctgctgctgctgctgctgctcatccccagaggatggacaggggcacttggggtcttcatccaagtcccccacccccgagtcatggaagtgcccagaagtgtccatcttggggcctggctgtattccctgcagcacaagcccccaccccaaagccaccctcgctccaaagatgtcctcaaagaaagccaggcatccaatctcccccaccagtatcttggctccagtcctctctttggcttgcttcggttctctggggctgcctggagtccagacgctgccactcaagaatgcattgtattgggcagggagggagagcaggaggggagcttggagaaagaagagggggtgaaagaactctctcaggaggtggtcctctaggagcgtgtgaggccaggctcagcttcactcctcgctggctcaat

SEQ ID NO: 14151 - RNA, 5239 nt, Homo sapiens
  source 1..5239: mol_type = other RNA
gctgggattacaggcatgagccaccgcacctggtcatcaataacaatccttttattattttttttaagatggagtctcgctctgtcgcccaggctggagcgcagtggcacaatcttggctccctgcaagctccgcctcccgggttcacaccattctcctgcctcagcctcccgagtagctgggactataggcgcatgccacgcctggctaattttttgtatttttagtacagacggggtttcaccgtgttagccaggatggtctcaatctcctgacctcgtgatccacctgcctcggcctcccaaagtgctgggattacaggtgtgagccaccgcgcccggcccagtaacaatctttatacacatctctggttgcactcatgtgtcacacacaacctttaccacaatcacatgctggaacttgtgtatccctacatgaccttggaaaatcgcttgaagtctcagaagcttagtttcctcatcagtaaattggggtaataaaatagcatgtatattggtgaagattcttgcttcaaagtagaggaaacaccttttgccacctggaaagcacttcctgaacattagttgtttatcgctcaggtattcgacatccaggaagtgctgagcatcctcccctgttaggggtacaatgggccggccctcatgctcacatgcagatgacacttatgggtacagcgacagaaaagcacacaagcctctctgctcactgaccaagctggagtggaagagacaggcgaggctcccgggaggaagtgacactgagctgagacctcaaaagatgaggaggcaaaaaaggtgagtgggagatcggaaggtgggaggctggccaggcagaggaagcagcgagtgtaagggatgagctgacgcaagagaacatgtttggagcctgagaggtgggtgtgagtgggcggtggcatacaaaaagtctggagaggtggcagagcagagaggccctaccccaaggccacagggagacagggaaggatttcaagcaggggagtgacaggcttggatttgtgtgtggggaaaactggtctggtctcagcgtggaggtggcatggagactgggagctgggagacccatgaggggaacacagaagtgacgttggtaaacatggtgagggctgaactaaagccaatgccgcttctgcgaccaagaatctgtcctcaggccctctagtagctgttgccttcctgaagcttgggatgcatatgcacaaagagagctctgtgtggctcacagattgtggacacctggttgacctcttgatgcctgcgtatcatgtctagctcctaagtctcccttctcctactacaacatcacacggtggccacgcctcccacaacacgcagtgggcatcatcagaggaacagcagctgatgggaaccatgcccccacagctccaagaggtctgaactcacacaccacaccccacactcttcttcttgggcttgctcagcaccttgtggggcacagcacccgaccctgcactctcaagtttccaggcgacaggagccctttaggcttcttggcaccaagggcacggctgggtccccaccaatgtcccatgataagagatgccaccagcagccaggctgcacagaacctacacggagtgaggggaagaggaggccaacacattctaggttggttaccactgggtggccttgtataatatctaaatatctaaacatctaaaatgagacaaggacagagatacgagaactgccccggactctctactccttaagtggagacccccttaacactctttttgattttattattattattttgagacagggtcttgctctgtcacacagattggagtgcagtggctcaatcacagctcactgtagcctcgacctccttggctcaagcaatactcccacctcagcctccaaagtagctgggactacaggcgcataccaccacataaggttaatcttttttttttttttttttttgtagagacagggttttgtcatgttggccaggctggcctcgaacttctgggctcaggcaatctgcctgccgcagcctcccaaagtgctgggattacaggcatgagccaccgtgtccggcaacactcttaatatgagtgacttcaaagcttttgaagcctctatccccgctggcagtggtgtgcccctgggctctccctagactaggctaaagcccctgccaaccactctcccagcaccctgcacttaccttttcatgacacccatcacttttagacttacaggttgaattgctgccttccttgctaggctgtaagttccccgatggacataactgcatctgcctggtgtgctgttgtttccctggtgtctgaacagagtcaggctcctgacaggcccccgctatttggagctgagtcaataggatgtgcaaactgagggagaggaaagggtggaggaaaactcgcagacctcagaggcctggggagaggaaaagtgtcttgctcaagtcacatactaggcaggaagagatcatggttcctgctcagaatctttgactctcagtcagggcctttcccactcactatactgtgctagaaagaggctacgaaacccacagaaaagtgttctatagttaaataagcttgaaaaactctggattaaacaaaatgaaaggagtttctttgccactggtcttttcagggcctttaacatgctcctgtgcccgtgcttctggaagaaggtcacacacagtactccatgctctctgaccctggaactctgcctgtgaggcggtctgaaacctccagcaccaccccccagctatgtgtcacaattatttattaaatgtgacacagcagagagatttgttgccattttttttagtggctaggaaaatccttttgtacaaataaaaataattcaaaaccccaatatatgaatgggataaaaatgcagctgctctggttgaagggggtactggggatccatctggagctgtcctttcactgctgctatgcaaagaacccttgcttcctgtagagcgcagttcgaaaatcactgatgcagaattggcacatgaggttgaagctaggaggcttctagtgctggctctgccatggactgttttaccctgggcaagtcatttagtctcactgggcttcagtttcccgtgtatacgataagtctgtcacactgtatgtttcttagagtcctgaactttcagctttgatatggtgaagagtacatttctatgactataaaagtctaactctaagattccatggcttaatattccaattctgggactgcctgtagctagcccaagctggtgcagcacgctagagcccaggctgttgaaggcagaattcattaactgcagtgcgctgcccaggggcactgggttcctgggataggggtgccaggttcctggggtgggtggaccgtgatcggcagccgctcagtgggacaagctgggagagggacccaggtctcctgactcctgctctatctttagatctccatagcaaccatcaccagggcaccaagctgaaggcacaggctgagtggctgcctgcaggaggagggaggggcgtttccttcccgtgcctcttcttttgctaggctcgatttttgagccaggaaaggggactgagaatgaagctgttcacagcaagaaaggcttggggccaatacaagacagtcgagggccccaccttgctctcaggatgtggtcaagtcatagaacccaagaccttcatgtgtcaggctcatggcactggaggaaaggcagaatcctcctccaaagagctctaagcctctcccgtgtccttccctacacactcaggagcccctaatccgagatggtgctgaggccacagttggagcccccattagatcctctaatcggaggggccagggaagctcctcccgactcttcccctgcccaactcctactcctcctggggctcagcctggacttggcttcctctgaagagtcctccctgactcccaggctggttgctcacctcctcagggcccctacagcccatcctccttctacatagtaggaggccaggaggagtgattaacctcatggggcagatgagaagtagaggttctgagcagtaaagacacttgcccaaggtcacctggcaaatgagcagcaggaccaggcctggactccgtgtcttctgattccagtctgtgctccttcctgggtcccagtagcaggctcatggcctaggctttggaagagaggccagggctagaagaggaaataggagtcctcagtgaggcctgcgcacagtaagcacctggctatgtctttggtgaactcagccgagccacagaccagtgcgaatggctttctccgacagcagctgaccagctctttaattaggtcctggcccaggtggccaaagtgggttttctcttggtaactccagggaagctgctctgaggagctctcctggctgagtacaaagaaggtacggacattccagaaacgggcctgctcttggaggaaggttttcaggtagatgctctcaaaggtcttgaagcaaccgaccagagtgacaaaagtctcgtcattctcattgtctgtgatgctctgcaggataggcaccatgggggccaggcccgtgcccgcagccagcaagaggagctcaccatactggtttggtttatagaagaaatctccgaaaggtcctcgccagaaagctgtgtctcctactctccaggactcaacataccgggacatcagccccatctggtagcactgtgactctggcccacgcagcaggctcctgtccttgctggcttgggctgcctcccaccttgccagatctcggtgatagaggtcaaacacacagggtgagcagccactgccgcagcactgggaaggcaagggttctgtgggccgtagctgcatccaggcttcctcagtgtcgtcgtcctcttccctctcagccatcatcagtggggcttgggcagcctagaaggaacaactgggtgctcttccagaacaggccaggctctatgagaccacgggcgcaggccctgctccttggccagcattttgtagagacagggtctcactatgttgccagtctggtctcgaactcctggcctcaagtgatcttctcatctcagtctcccaaagtgctgagattacaggcatgagccaccatgtctggccctactcgcctgcgcttcacctcacgtgaggattttccaggttcctcccagtctct

SEQ ID NO: 14152 - RNA, 5476 nt, Homo sapiens
  source 1..5476: mol_type = other RNA
gctgggattacaggcatgagccaccgcacctggtcatcaataacaatccttttattattttttttaagatggagtctcgctctgtcgcccaggctggagcgcagtggcacaatcttggctccctgcaagctccgcctcccgggttcacaccattctcctgcctcagcctcccgagtagctgggactataggcgcatgccacgcctggctaattttttgtatttttagtacagacggggtttcaccgtgttagccaggatggtctcaatctcctgacctcgtgatccacctgcctcggcctcccaaagtgctgggattacaggtgtgagccaccgcgcccggcccagtaacaatctttatacacatctctggttgcactcatgtgtcacacacaacctttaccacaatcacatgctggaacttgtgtatccctacatgaccttggaaaatcgcttgaagtctcagaagcttagtttcctcatcagtaaattggggtaataaaatagcatgtatattggtgaagattcttgcttcaaagtagaggaaacaccttttgccacctggaaagcacttcctgaacattagttgtttatcgctcaggtattcgacatccaggaagtgctgagcatcctcccctgttaggggtacaatgggccggccctcatgctcacatgcagatgacacttatgggtacagcgacagaaaagcacacaagcctctctgctcactgaccaagctggagtggaagagacaggcgaggctcccgggaggaagtgacactgagctgagacctcaaaagatgaggaggcaaaaaaggtgagtgggagatcggaaggtgggaggctggccaggcagaggaagcagcgagtgtaagggatgagctgacgcaagagaacatgtttggagcctgagaggtgggtgtgagtgggcggtggcatacaaaaagtctggagaggtggcagagcagagaggccctaccccaaggccacagggagacagggaaggatttcaagcaggggagtgacaggcttggatttgtgtgtggggaaaactggtctggtctcagcgtggaggtggcatggagactgggagctgggagacccatgaggggaacacagaagtgacgttggtaaacatggtgagggctgaactaaagccaatgccgcttctgcgaccaagaatctgtcctcaggccctctagtagctgttgccttcctgaagcttgggatgcatatgcacaaagagagctctgtgtggctcacagattgtggacacctggttgacctcttgatgcctgcgtatcatgtctagctcctaagtctcccttctcctactacaacatcacacggtggccacgcctcccacaacacgcagtgggcatcatcagaggaacagcagctgatgggaaccatgcccccacagctccaagaggtctgaactcacacaccacaccccacactcttcttcttgggcttgctcagcaccttgtggggcacagcacccgaccctgcactctcaagtttccaggcgacaggagccctttaggcttcttggcaccaagggcacggctgggtccccaccaatgtcccatgataagagatgccaccagcagccaggctgcacagaacctacacggagtgaggggaagaggaggccaacacattctaggttggttaccactgggtggccttgtataatatctaaatatctaaacatctaaaatgagacaaggacagagatacgagaactgccccggactctctactccttaagtggagacccccttaacactctttttgattttattattattattttgagacagggtcttgctctgtcacacagattggagtgcagtggctcaatcacagctcactgtagcctcgacctccttggctcaagcaatactcccacctcagcctccaaagtagctgggactacaggcgcataccaccacataaggttaatcttttttttttttttttttttgtagagacagggttttgtcatgttggccaggctggcctcgaacttctgggctcaggcaatctgcctgccgcagcctcccaaagtgctgggattacaggcatgagccaccgtgtccggcaacactcttaatatgagtgacttcaaagcttttgaagcctctatccccgctggcagtggtgtgcccctgggctctccctagactaggctaaagcccctgccaaccactctcccagcaccctgcacttaccttttcatgacacccatcacttttagacttacaggttgaattgctgccttccttgctaggctgtaagttccccgatggacataactgcatctgcctggtgtgctgttgtttccctggtgtctgaacagagtcaggctcctgacaggcccccgctatttggagctgagtcaataggatgtgcaaactgagggagaggaaagggtggaggaaaactcgcagacctcagaggcctggggagaggaaaagtgtcttgctcaagtcacatactaggcaggaagagatcatggttcctgctcagaatctttgactctcagtcagggcctttcccactcactatactgtgctagaaagaggctacgaaacccacagaaaagtgttctatagttaaataagcttgaaaaactctggattaaacaaaatgaaaggagtttctttgccactggtcttttcagggcctttaacatgctcctgtgcccgtgcttctggaagaaggtcacacacagtactccatgctctctgaccctggaactctgcctgtgaggcggtctgaaacctccagcaccaccccccagctatgtgtcacaattatttattaaatgtgacacagcagagagatttgttgccattttttttagtggctaggaaaatccttttgtacaaataaaaataattcaaaaccccaatatatgaatgggataaaaatgcagctgctctggttgaagggggtactggggatccatctggagctgtcctttcactgctgctatgcaaagaacccttgcttcctgtagagcgcagttcgaaaatcactgatgcagaattggcacatgaggttgaagctaggaggcttctagtgctggctctgccatggactgttttaccctgggcaagtcatttagtctcactgggcttcagtttcccgtgtatacgataagtctgtcacactgtatgtttcttagagtcctgaactttcagctttgatatggtgaagagtacatttctatgactataaaagtctaactctaagattccatggcttaatattccaattctgggactgcctgtagctagcccaagctggtgcagcacgctagagcccaggctgttgaaggcagaattcattaactgcagtgcgctgcccaggggcactgggttcctgggataggggtgccaggttcctggggtgggtggaccgtgatcggcagccgctcagtgggacaagctgggagagggacccaggtctcctgactcctgctctatctttagatctccatagcaaccatcaccagggcaccaagctgaaggcacaggctgagtggctgcctgcaggaggagggaggggcgtttccttcccgtgcctcttcttttgctaggctcgatttttgagccaggaaaggggactgagaatgaagctgttcacagcaagaaaggcttggggccaatacaagacagtcgagggccccaccttgctctcaggatgtggtcaagtcatagaacccaagaccttcatgtgtcaggctcatggcactggaggaaaggcagaatcctcctccaaagagctctaagcctctcccgtgtccttccctacacactcaggagcccctaatccgagatggtgctgaggccacagttggagcccccattagatcctctaatcggaggggccagggaagctcctcccgactcttcccctgcccaactcctactcctcctggggctcagcctggacttggcttcctctgaagagtcctccctgactcccaggctggttgctcacctcctcagggcccctacagcccatcctccttctacatagtaggaggccaggaggagtgattaacctcatggggcagatgagaagtagaggttctgagcagtaaagacacttgcccaaggtcacctggcaaatgagcagcaggaccaggcctggactccgtgtcttctgattccagtctgtgctccttcctgggtcccagtagcaggctcatggcctaggctttggaagagaggccagggctagaagaggaaataggagtcctcagtgaggcctgcgcacagtaagcacctggctatgtctttggtgaactcagccgagccacagaccagtgcgaatggctttctccgacagcagctgaccagctctttaattaggtcctggcccaggtggccaaagtgggttttctcttggtaactccagggaagctgctctgaggagctctcctggctgagtacaaagaaggtacggacattccagaaacgggcctgctcttggaggaaggttttcaggtagatgctctcaaaggtcttgaagcaaccgaccagagtgacaaaagtctcgtcattctcattgtctgtgatgctctgcaggataggcaccatgggggccaggcccgtgcccgcagccagcaagaggagctcaccatactggtttggtttatagaagaaatctccgaaaggtcctcgccagaaagctgtgtctcctactctccaggactcaacataccgggacatcagccccatctggtagcacttaattaacacttcaaagtatccttctgcgttggcagggctgatgggcgtataggctctctgaatttctaagtcatctactatccctcgtaggatgaggtgctggccgggccgcaggccaagctggctgttcccgggtagagcaaaccggacacggtaggtgtccttagtgagcctgtccatggcaatgatgcagaaggccacgaaggtctctgggttcagcttggaggggcagctctgtgactctggcccacgcagcaggctcctgtccttgctggcttgggctgcctcccaccttgccagatctcggtgatagaggtcaaacacacagggtgagcagccactgccgcagcactgggaaggcaagggttctgtgggccgtagctgcatccaggcttcctcagtgtcgtcgtcctcttccctctcagccatcatcagtggggcttgggcagcctagaaggaacaactgggtgctcttccagaacaggccaggctctatgagaccacgggcgcaggccctgctccttggccagcattttgtagagacagggtctcactatgttgccagtctggtctcgaactcctggcctcaagtgatcttctcatctcagtctcccaaagtgctgagattacaggcatgagccaccatgtctggccctactcgcctgcgcttcacctcacgtgaggattttccaggttcctcccagtctct

SEQ ID NO: 14153 - RNA, 5327 nt, Homo sapiens
  source 1..5327: mol_type = other RNA
gctgggattacaggcatgagccaccgcacctggtcatcaataacaatccttttattattttttttaagatggagtctcgctctgtcgcccaggctggagcgcagtggcacaatcttggctccctgcaagctccgcctcccgggttcacaccattctcctgcctcagcctcccgagtagctgggactataggcgcatgccacgcctggctaattttttgtatttttagtacagacggggtttcaccgtgttagccaggatggtctcaatctcctgacctcgtgatccacctgcctcggcctcccaaagtgctgggattacaggtgtgagccaccgcgcccggcccagtaacaatctttatacacatctctggttgcactcatgtgtcacacacaacctttaccacaatcacatgctggaacttgtgtatccctacatgaccttggaaaatcgcttgaagtctcagaagcttagtttcctcatcagtaaattggggtaataaaatagcatgtatattggtgaagattcttgcttcaaagtagaggaaacaccttttgccacctggaaagcacttcctgaacattagttgtttatcgctcaggtattcgacatccaggaagtgctgagcatcctcccctgttaggggtacaatgggccggccctcatgctcacatgcagatgacacttatgggtacagcgacagaaaagcacacaagcctctctgctcactgaccaagctggagtggaagagacaggcgaggctcccgggaggaagtgacactgagctgagacctcaaaagatgaggaggcaaaaaaggtgagtgggagatcggaaggtgggaggctggccaggcagaggaagcagcgagtgtaagggatgagctgacgcaagagaacatgtttggagcctgagaggtgggtgtgagtgggcggtggcatacaaaaagtctggagaggtggcagagcagagaggccctaccccaaggccacagggagacagggaaggatttcaagcaggggagtgacaggcttggatttgtgtgtggggaaaactggtctggtctcagcgtggaggtggcatggagactgggagctgggagacccatgaggggaacacagaagtgacgttggtaaacatggtgagggctgaactaaagccaatgccgcttctgcgaccaagaatctgtcctcaggccctctagtagctgttgccttcctgaagcttgggatgcatatgcacaaagagagctctgtgtggctcacagattgtggacacctggttgacctcttgatgcctgcgtatcatgtctagctcctaagtctcccttctcctactacaacatcacacggtggccacgcctcccacaacacgcagtgggcatcatcagaggaacagcagctgatgggaaccatgcccccacagctccaagaggtctgaactcacacaccacaccccacactcttcttcttgggcttgctcagcaccttgtggggcacagcacccgaccctgcactctcaagtttccaggcgacaggagccctttaggcttcttggcaccaagggcacggctgggtccccaccaatgtcccatgataagagatgccaccagcagccaggctgcacagaacctacacggagtgaggggaagaggaggccaacacattctaggttggttaccactgggtggccttgtataatatctaaatatctaaacatctaaaatgagacaaggacagagatacgagaactgccccggactctctactccttaagtggagacccccttaacactctttttgattttattattattattttgagacagggtcttgctctgtcacacagattggagtgcagtggctcaatcacagctcactgtagcctcgacctccttggctcaagcaatactcccacctcagcctccaaagtagctgggactacaggcgcataccaccacataaggttaatcttttttttttttttttttttgtagagacagggttttgtcatgttggccaggctggcctcgaacttctgggctcaggcaatctgcctgccgcagcctcccaaagtgctgggattacaggcatgagccaccgtgtccggcaacactcttaatatgagtgacttcaaagcttttgaagcctctatccccgctggcagtggtgtgcccctgggctctccctagactaggctaaagcccctgccaaccactctcccagcaccctgcacttaccttttcatgacacccatcacttttagacttacaggttgaattgctgccttccttgctaggctgtaagttccccgatggacataactgcatctgcctggtgtgctgttgtttccctggtgtctgaacagagtcaggctcctgacaggcccccgctatttggagctgagtcaataggatgtgcaaactgagggagaggaaagggtggaggaaaactcgcagacctcagaggcctggggagaggaaaagtgtcttgctcaagtcacatactaggcaggaagagatcatggttcctgctcagaatctttgactctcagtcagggcctttcccactcactatactgtgctagaaagaggctacgaaacccacagaaaagtgttctatagttaaataagcttgaaaaactctggattaaacaaaatgaaaggagtttctttgccactggtcttttcagggcctttaacatgctcctgtgcccgtgcttctggaagaaggtcacacacagtactccatgctctctgaccctggaactctgcctgtgaggcggtctgaaacctccagcaccaccccccagctatgtgtcacaattatttattaaatgtgacacagcagagagatttgttgccattttttttagtggctaggaaaatccttttgtacaaataaaaataattcaaaaccccaatatatgaatgggataaaaatgcagctgctctggttgaagggggtactggggatccatctggagctgtcctttcactgctgctatgcaaagaacccttgcttcctgtagagcgcagttcgaaaatcactgatgcagaattggcacatgaggttgaagctaggaggcttctagtgctggctctgccatggactgttttaccctgggcaagtcatttagtctcactgggcttcagtttcccgtgtatacgataagtctgtcacactgtatgtttcttagagtcctgaactttcagctttgatatggtgaagagtacatttctatgactataaaagtctaactctaagattccatggcttaatattccaattctgggactgcctgtagctagcccaagctggtgcagcacgctagagcccaggctgttgaaggcagaattcattaactgcagtgcgctgcccaggggcactgggttcctgggataggggtgccaggttcctggggtgggtggaccgtgatcggcagccgctcagtgggacaagctgggagagggacccaggtctcctgactcctgctctatctttagatctccatagcaaccatcaccagggcaccaagctgaaggcacaggctgagtggctgcctgcaggaggagggaggggcgtttccttcccgtgcctcttcttttgctaggctcgatttttgagccaggaaaggggactgagaatgaagctgttcacagcaagaaaggcttggggccaatacaagacagtcgagggccccaccttgctctcaggatgtggtcaagtcatagaacccaagaccttcatgtgtcaggctcatggcactggaggaaaggcagaatcctcctccaaagagctctaagcctctcccgtgtccttccctacacactcaggagcccctaatccgagatggtgctgaggccacagttggagcccccattagatcctctaatcggaggggccagggaagctcctcccgactcttcccctgcccaactcctactcctcctggggctcagcctggacttggcttcctctgaagagtcctccctgactcccaggctggttgctcacctcctcagggcccctacagcccatcctccttctacatagtaggaggccaggaggagtgattaacctcatggggcagatgagaagtagaggttctgagcagtaaagacacttgcccaaggtcacctggcaaatgagcagcaggaccaggcctggactccgtgtcttctgattccagtctgtgctccttcctgggtcccagtagcaggctcatggcctaggctttggaagagaggccagggctagaagaggaaataggagtcctcagtgaggcctgcgcacagtaagcacctggctatgtctttggtgaactcagccgagccacagaccagtgcgaatggctttctccgacagcagctgaccagctctttaattaggtcctggcccaggtggccaaagtgggttttctcttggtaactccagggaagctgctctgaggagctctcctggctgagtacaaagaaggtacggacattccagaaacgggcctgctcttggaggaaggttttcaggtagatgctctcaaaggtcttgaagcaaccgaccagagtgacaaaagtctcgtcattctcattgtctgtgatgctctgcaggataggcaccatgggggccaggcccgtgcccgcagccagcaagaggagctcaccatactggtttggtttatagaagaaatctccgaaaggtcctcgccagaaagctgtgtctcctactctccaggactcaacataccgggacatcagccccatctggtagcacttaattaacacttcaaagtatccttctgcgttggcagggctgatgggcgtataggctctctgaatttctaagtcatctactatccctctgtgactctggcccacgcagcaggctcctgtccttgctggcttgggctgcctcccaccttgccagatctcggtgatagaggtcaaacacacagggtgagcagccactgccgcagcactgggaaggcaagggttctgtgggccgtagctgcatccaggcttcctcagtgtcgtcgtcctcttccctctcagccatcatcagtggggcttgggcagcctagaaggaacaactgggtgctcttccagaacaggccaggctctatgagaccacgggcgcaggccctgctccttggccagcattttgtagagacagggtctcactatgttgccagtctggtctcgaactcctggcctcaagtgatcttctcatctcagtctcccaaagtgctgagattacaggcatgagccaccatgtctggccctactcgcctgcgcttcacctcacgtgaggattttccaggttcctcccagtctct

SEQ ID NO: 14154 - RNA, 380 nt, Homo sapiens
  source 1..380: mol_type = other RNA
gctgggattacaggcatgagccaccgcaccttgcctctcttttacgttttaaatgtggttcctagacaaccttaattttgtagcttgtacccaagtttgtgatgtcaattgccaagactaaggaatgaaacgtcttcatacgaggtcatcccggagccaactcattgcctgctttttttctgtgtatgttggtggtgtggcggggacaggattgataagcactgtcatcacagcactccagctggctgcagtctccgttgctgccaccaaccacagcgatgtgagccacagtggcacaggctgcagcatccagcgtgtagcaggtggcttctccctctggtcctctaagctgggaacagagcagctggtcaggaagacac

SEQ ID NO: 14155 - RNA, 1846 nt, Homo sapiens
  source 1..1846: mol_type = other RNA
gctgggattacaggcatgagccaccgcaccttgcctctcttttacgttttaaatgtggttcctagacaaccttaattttgtagcttgtacccaagtttgtgatgtcaattgccaagactaaggaatgaaacgtcttcatacgaggtcatcccggagccaactcattgcctgctttttttctgtgtatgttggtggtgtggcggggacaggattgataagcactgtcatcacagctctatgtgaaggggtgacagacataaaaaccaaaatagtcttccagaagcttcggagttccagagggaggtgagtggacctctctccagcagcagaaaatccccaatcactgggagggaccagccccctgccagaagtgaagatggatagtctctctcctgtttggaaatactgagcctgagctcgttccgcaacatctaggtcatgttggtctggtcctgatttccagcagggcagtgctgagcttcaggtgcaagtttaggactcagcagaaccacctgctgacatcaaaccaacgctccactggagtcctgagaatacaaggctgaaaaggctagtgcactgcgctcaagcggccatggccttcctgtgcctgtggattgcatcaagcaccttcgtggcctttttatcctgggcctgggatgcactctcatggtcctgcccagcctggagctccaggcaaccctaccaccagatcggggccagccttcagggcaatgagtgttggcacatccatttgtaaatcttagctttgtgcatccatttctaaatcttagccagtcgccttcacctgaaagctagctagctctagcctgatggtgtctgtctgcaccctacccttgtcgtggagatgctgctgcttttgttccctgccctcacatggctgagcagcctccccacgggaaactcatggggccagaaggctggcccctggcttggggaggacagcaaagcccgtgcagcctgcctgcagctggttctgcatcattgccttctgtagctcaggaggagttacccttgccctcctgtctcccagactactccggctgctccccagcatcctggcattattgaagtgacagaaagcttctggctgcatctgagagctgtttggatattttaaccacacataaatgcactgagaggcaactaggttaataaataggcctactagaggcgaagcccaagcataaaattgagggagaagccacccggaaaatgcaagaatccccagatccgatgatcagatgtgagagaatgcacacttggtgctctctaaaggcctagaactaaaaggcaacagctccctcgtgactgtagtgttgtgtgaaagaaaagtagaatcccaggacccaaactcactatgctgaagggaaagttaagcttgggaactgagtcactgataatgttttcctaaacagctgtaatttcacaacctggcttcacagcctcattctctctgctccctcttttcacaagcttgctttatcatccgtagaatgcagatttactgtgctcgaggtaatgcatagctgacattctcctctactccatcttttcacatgtgaaatgtagatttactaaagctagacagagctgcacaagatgtaagcattggtttcactgcctcacctcttcccttttcccccctcctgcttgctctttcccctttaaatactgaagttcacaaagccccctttaggaaaagcagaggtcacagatgcccctgttgtcagaggtatgtgaaccagagcaaatccatcttaaataggagctgggtaaaatgaggctgagacctactgggctgcattcccagatggttaagccattc

SEQ ID NO: 14156 - RNA, 650 nt, Homo sapiens
  source 1..650: mol_type = other RNA
gctgggattacaggcatgagccaccgcacgcggccaattgtaaacttcttgaggttgtcaccagaagcagatgctggcatcatgcttcttgtacagcctagaaaggcctgtctgtctagattcttcttggcatctctgagcatggatttcattctggatatggggcaggatgctctctggaatgagggtctttagacctgtttctttgttctgatgggaccccagagaggacatcacgctttgtaactggttcttcaaggggagaagcaaatgtgtccctgaaaacttcagctgccgcgtttggcaccaggtttgattgacaaggactggcggagggaaagcgcggaggctgggctgggggccgcaggccgaggcagagacaaagaggtttcgcctgtccccgagagtggaagggcccctgggggtaactagcctttgagctcaaaggggcatttcgtgaggtcgccttttggttcggagagcgcgcggcgatcgggtggagggggcctggcgggaagaaagctggggcggggaaggggcgcgggccgaggtgggagcggagctgcagtcacgtggccgcccgccgccgcggagttggggctgttcttccgggttggaggcgcagcgccgcggggcccaagcccgggtct

SEQ ID NO: 14157 - RNA, 2385 nt, Homo sapiens
  source 1..2385: mol_type = other RNA
gctgggattacaggcatgagccaccgcacgtggcctagatgaaagtttttaaaagcctgggctaataaaatcatccaccaatcatttttcttatggttaaagcagccaaaaagctgtcacagcatttttgagatgagaacataaggcttgtgtggctttatgatagatgctgttagtcattttatttgattaagcccttggtcagtcatctataccttaattaatattttgttcttatagaaaaatacaatccattttatgagtttctagaaataaataatggagaaaaatagatactacctgttcctaatggtctctctggaaattacagcttttgcctaggaagatacacatatagaatataatttaagttcaaaatatatttcattatattctatcccttttaattttttgtttgtttctttgagacggagtcttgctctgtccacccaggctggagtgcagtggcacgatctctgctcactgcaacctccgcctcctgggttcaaccaattctcctgcctcagcctcccgagtagctgggactacaggtgtgcgccaccacacctggctaatttttgtatttttagtagagacagggtttcaccatgctggccaggctggtctcgaactcccaacctcaggcgatccatctgcctcagcctcccaaagtgctgggattaaaggcgtgagccactgtgcccagccttttttttttttttttttttccgagacaagagtctcactctgttgcccaggctggagcacagcggtgcaatcttggctcactacaacctccacctcctgggtttaggcgattctcctgcctcagcctcccaaatagctgggattacaggcacatgccaccacacctggctaatttttgtatttttagtagcgacggggtttcgccatgttggccaggctggtctcgaactcctgacctcaggcgatccacttcccgacctcaggtgatccgcctgcctcggcctctaaaagtgctgcaattacaggcataagccactgtgcctggccctatcccttttaattttctaagtgaccagtaataaacaatgatttgtttattactaggtagcaggagaaaaactttttagtcacttttccagctaagaatttcatttaaagatacctatgacatatcttgtggtactaagaatattagagaactggaaatccagtttttttgtggttttttaagaaagagaatctgactccattgcccagcttggagagcagtggtgcaatagctggggctacaggcgtgagccaccacaccaggcctggaaacccagttttaatttgtgaactacaaatggttggcaactgattccttaattgttattgcaggagtaggcccaacatgagtccatatgtagcccttctctggtctggtgggaactgtgggaaatggtgatgaccgtgacttgaaatactcagaaggtgcatgacaaacaaattccaagtattccatcttccttggaagatcttcctctggccctatgatataggaggcgggatcaaattggtctctggggctagagagggtaggaatgagccacgtcagtgctgcactcttctcgcaatactggtcctggataaaacctctgatttgagcatagtagggctttccatcttgttcatcaatcacagaaacaacatcaccaatttggtaatatactcccttgtagaagattgattctgcagtgattatagtggaaactgactcaggagctttgatgggatttttcaatttaaatatatgtcttctcccttttcctttggtggagactttcttttcagcagccggagcagatttgtatttagtgtttctgagccgagcagacctcctgtgaatttcctgcttactctgcttgccgcccccgcccccgttgctctgcggaggggtggcggaggtgctggcgaaggtcgccgcgccgaagccgccgccgccgctgcccccagtccctccagccgcccccgagcctgcgcccccgctgcccgcgccgccccggccagtgcaatgatggcagaggatctccccctgcgctcccttcttccacatggaggacgacgtggtcttgcatacgctgcaggtgggcttcaggcccagcggcatggtggccggctcgggcggcccccgcgggcgcagagacacgggaatggcggacggtagcccggccgccccctggtcggcccgccactcccggcgataggaagagcggtgagagcgtcggcacggagctgccggtgaaaggaccaggccgctggcgctgccccgtggaggcgggaagcgggttccgccggctccgcaggcggaggccaggattccctggcccgaggcactgggaagcaggactgggaaag

SEQ ID NO: 14158 - RNA, 3994 nt, Homo sapiens
  source 1..3994: mol_type = other RNA
gctgggattacaggcatgagccaccgcacgtggcctagatgaaagtttttaaaagcctgggctaataaaatcatccaccaatcatttttcttatggttaaagcagccaaaaagctgtcacagcatttttgagatgagaacataaggcttgtgtggctttatgatagatgctgttagtcattttatttgattaagcccttggtcagtcatctataccttaattaatattttgttcttatagaaaaatacaatccattttatgagtttctagaaataaataatggagaaaaatagatactacctgttcctaatggtctctctggaaattacagcttttgcctaggaagatacacatatagaatataatttaagttcaaaatatatttcattatattctatcccttttaattttttgtttgtttctttgagacggagtcttgctctgtccacccaggctggagtgcagtggcacgatctctgctcactgcaacctccgcctcctgggttcaaccaattctcctgcctcagcctcccgagtagctgggactacaggtgtgcgccaccacacctggctaatttttgtatttttagtagagacagggtttcaccatgctggccaggctggtctcgaactcccaacctcaggcgatccatctgcctcagcctcccaaagtgctgggattaaaggcgtgagccactgtgcccagccttttttttttttttttttttccgagacaagagtctcactctgttgcccaggctggagcacagcggtgcaatcttggctcactacaacctccacctcctgggtttaggcgattctcctgcctcagcctcccaaatagctgggattacaggcacatgccaccacacctggctaatttttgtatttttagtagcgacggggtttcgccatgttggccaggctggtctcgaactcctgacctcaggcgatccacttcccgacctcaggtgatccgcctgcctcggcctctaaaagtgctgcaattacaggcataagccactgtgcctggccctatcccttttaattttctaagtgaccagtaataaacaatgatttgtttattactaggtagcaggagaaaaactttttagtcacttttccagctaagaatttcatttaaagatacctatgacatatcttgtggtactaagaatattagagaactggaaatccagtttttttgtggttttttaagaaagagaatctgactccattgcccagcttggagagcagtggtgcaatagctggggctacaggcgtgagccaccacaccaggcctggaaacccagttttaatttgtgaactacaaatggttggcaactgattccttaattgttattgcaggagtaggcccaacatgagtccatatgtagcccttctctggtctggtgggaactgtgggaaatggtgatgaccgtgacttgaaatactcagaaggtgcatgacaaacaaattccaagtattccatcttccttggaagatcttcctctggccctatgatataggaggcgggatcaaattggtctctggggctagagagggtaggaatgagccacgtcagtgctgcactcttctcgcaatactggtcctggataaaacctctgatttgagcatagtagggctttccatcttgttcatcaatcacagaaacaacatcaccaatttggtaatatactcccttgtagaagattgattctgcagtgattatagtggaaactgactcaggagctttgatgggctatgaaaatacaaaaaacattagcacattcatagtatgtatgtgtctacaggcattttcccagccctatgagagttctgcaatttgagaagtactaaaatgtattgtttggtgacaagaactgcaataaaaagataaatgattttctgaatgttgtggcaaagcagtctatttccactgcaatttctgctactattagcttaaaaattgctgagacaaaggacaaccttctgattatgctgctgagatctaatgcaaagtcctctcagagcttcactacacataaacattccagttataaaaatgtacctgctctaatagcctgagcatgacagaatgcaagtaacagaaaatgtacagatgaatacaaagtgaaaaagtgtctcctcaaagacatttcccaactcaactatggaactagccataatactcaacataggttttctagcaagctgaaactaaggctttagaaactttgagagttcttagtaatttgctaccatccaaccatttttgagatctctactaaagcttcaatacatacttttatgccacaacatagaaagtaggcctccccagatgtgtcttgcttagtaccattgaagaaaggttgcagagaaacgataatgaaataattgctgagaacacggtataccatacttaaaaggaaaaaaatgtgcatatgtgatacaaatatcaataacatgttttgtgtaatcaacaaatgcctcacttaactataaaaatcttaaataaattagaagcaactagtctgaataagaaaatactttggggaagggaacatcacacactggggcctgtcggagatgggggccaaggggagggagagcattaggacaaatatctaatgcatgcggggcttaaaacctagatgatgggttgataggtgcagcaaaccaccatggcacgtatacctatgtaacaaacctgcacattctgcacatgtatcccagaacttaaagtaaaattaaaaaaaattcattaaattaaattaaaaaaaaaaaaagaaaatagtctgccatctgcataagtctactgcagggtccctttgtgttttagaaataaatatggccaacttcagaaacgtctttacgggtaagtgaaacattcctgttctgaaagaaaagaatatcatactgagacttaaaaaaatagtccataatgcactgtccactgtgtttgaacattatcccttgtttataaaaactgagaatttaattgcaataaaaatatgctttcaactacttccagcacaggtctttcaacaatctcttttcttagagcagaagaggagataaggcttagcaaaatttttgactcatattcatcaaatacatcatcatcataagtcagtaagatacattttctggggctttaataacaaataaatatgcaaatgatgagttctagtgttaatatttacttagatttttaaagaatgaaaaaaaaaagttttcttagtgtacctggccatatcaagaaccataatctctcctcttcctttccatagagaaccccaaaaaatgggctcaaggttgatgtttcttttaaacccatattttatattttccaggggaaaaaataaaagatttttcaatttaaatatatgtcttctcccttttcctttggtggagactttcttttcagcagccggagcagatttgtatttagtgtttctgagccgagcagacctcctgtgaatttcctgcttactctgcttgccgcccccgcccccgttgctctgcggaggggtggcggaggtgctggcgaaggtcgccgcgccgaagccgccgccgccgctgcccccagtccctccagccgcccccgagcctgcgcccccgctgcccgcgccgccccggccagtgcaatgatggcagaggatctccccctgcgctcccttcttccacatggaggacgacgtggtcttgcatacgctgcaggtgggcttcaggcccagcggcatggtggccggctcgggcggcccccgcgggcgcagagacacgggaatggcggacggtagcccggccgccccctggtcggcccgccactcccggcgataggaagagcggtgagagcgtcggcacggagctgccggtgaaaggaccaggccgctggcgctgccccgtggaggcgggaagcgggttccgccggctccgcaggcggaggccaggattccctggcccgaggcactgggaagcaggactgggaaag

SEQ ID NO: 14159 - RNA, 1923 nt, Homo sapiens
  source 1..1923: mol_type = other RNA
gctgggattacaggcatgagccaccgcacgtggcctagatgaaagtttttaaaagcctgggctaataaaatcatccaccaatcatttttcttatggttaaagcagccaaaaagctgtcacagcatttttgagatgagaacataaggcttgtgtggctttatgatagatgctgttagtcattttatttgattaagcccttggtcagtcatctataccttaattaatattttgttcttatagaaaaatacaatccattttatgagtttctagaaataaataatggagaaaaatagatactacctgttcctaatggtctctctggaaattacagcttttgcctaggaagatacacatatagaatataatttaagttcaaaatatatttcattatattctatcccttttaattttttgtttgtttctttgagacggagtcttgctctgtccacccaggctggagtgcagtggcacgatctctgctcactgcaacctccgcctcctgggttcaaccaattctcctgcctcagcctctaaaagtgctgcaattacaggcataagccactgtgcctggccctatcccttttaattttctaagtgaccagtaataaacaatgatttgtttattactaggtagcaggagaaaaactttttagtcacttttccagctaagaatttcatttaaagatacctatgacatatcttgtggtactaagaatattagagaactggaaatccagtttttttgtggttttttaagaaagagaatctgactccattgcccagcttggagagcagtggtgcaatagctggggctacaggcgtgagccaccacaccaggcctggaaacccagttttaatttgtgaactacaaatggttggcaactgattccttaattgttattgcaggagtaggcccaacatgagtccatatgtagcccttctctggtctggtgggaactgtgggaaatggtgatgaccgtgacttgaaatactcagaaggtgcatgacaaacaaattccaagtattccatcttccttggaagatcttcctctggccctatgatataggaggcgggatcaaattggtctctggggctagagagggtaggaatgagccacgtcagtgctgcactcttctcgcaatactggtcctggataaaacctctgatttgagcatagtagggctttccatcttgttcatcaatcacagaaacaacatcaccaatttggtaatatactcccttgtagaagattgattctgcagtgattatagtggaaactgactcaggagctttgatgggatttttcaatttaaatatatgtcttctcccttttcctttggtggagactttcttttcagcagccggagcagatttgtatttagtgtttctgagccgagcagacctcctgtgaatttcctgcttactctgcttgccgcccccgcccccgttgctctgcggaggggtggcggaggtgctggcgaaggtcgccgcgccgaagccgccgccgccgctgcccccagtccctccagccgcccccgagcctgcgcccccgctgcccgcgccgccccggccagtgcaatgatggcagaggatctccccctgcgctcccttcttccacatggaggacgacgtggtcttgcatacgctgcaggtgggcttcaggcccagcggcatggtggccggctcgggcggcccccgcgggcgcagagacacgggaatggcggacggtagcccggccgccccctggtcggcccgccactcccggcgataggaagagcggtgagagcgtcggcacggagctgccggtgaaaggaccaggccgctggcgctgccccgtggaggcgggaagcgggttccgccggctccgcaggcggaggccaggattccctggcccgaggcactgggaagcaggactgggaaag

SEQ ID NO: 14160 - RNA, 5889 nt, Homo sapiens
  source 1..5889: mol_type = other RNA
gctgggattacaggcatgagccaccgcactcagcctggcagttttaaacgaatgaattcatctgtaagcttttgaatggaaaaaccaaagtagaaagaaacatattgtcttacattattctacaaatcaaaacttttaaaaatcaaattgtctttcttgtattaagaacaaaccgcaagtgcctgatcatctactttatttccacgaggcagaaatacagttatgcagctgatgtcagggaaggcggagaatttcctcagccatccatgaagaaagataaggggccttatccactggctgtctaatcttataaagatctcatgcaaatttggtggacatagggcacaattctctatccttgaagaacattttccaaagcacagatgtttttctcttaattgtgaatgctgactgacttgtccatatcctttctcagtgctcagcagatggtacgatttgggactcgcttgttccctataacgtggggctgatgttctttgctacgtggaaaacacatctttggtgagacagaaatgaatcaatattacacaaaaatgtttccatttctggaatttccctgagataaaaatatctttctggctttgggtatacataagtgaccgtgcagacacttagtaaaagagaaaacagattttcaatacttcgtggtgatggtgactatacgggattataagtagttaaaggttttcctgttgcatcattttggaaacaaaaagctgactcattttctggttaatgcttcaatattttcattagggagtttctataaagtttttatctgaatcacagaaagtacaattatttcagaggtaggataaaattttttctgtcataaacagcactgtgtactaaaacctgctatgagtttaacaaatcacctagaagcctaatgctcaagaatgcaatatatcaagtaaaacactgaaaagttcaactagtttagataatgcaagtatggaaatgcaagattgactaaaacttttaaatattatcactcttattaacatgctaatttaattcattttactggagtattttaatttcctggcaattgaatagcactttttactacaaatatttcatcatttggataaacatattcttttatttaccatttgtcaggttttgtatgctaaattgcaactgcttatatacactcatcaagtatctcaaggataaattaaaattcttagtaaaaatccaactgaccggtacagaccacaaaaagtactattttaagcctttgggggcttaaaaattgtgtgtgtgtgtgtgtgtgtgtgtgtattcacatggtgggagaaaaagaactttccagataattgtgaatggcatactattatataagagtttaaaacgcaatatttctgtacgatcaaagttcttaactcatgctttttttttttttttttttttttgagacggggtttcgttcttgttgcccaggctgcagtgcagtggtacaatctcagctcactgcaacctctgcctcccaggttccagcgattctcctgccttagcctcccaagtagctgggattacaggtgcctgccaccacatctggctaatcttgtgtatttttagtagcagtggggtttcaccacgttggccaggctggtctcgaactcctcacctcaagtgatcctcccacctccgcctcccaaagttctgggcttacaagcataagccaccgcacccaccccatgctttactcttaaactaattttgagttgtatatgaaaggcctaataatcagaaaaaggctatttcttaacttaacttgctcaaatattttgagcctccaaatctggaaaataatgttgaagtttgaaactgatgccgtgcctactctagggagcacagtactgaactgctgcttccttgcttctcttggtgaatgcacattgagtgccttgtcatgctctgaacccaccactgctagggacagctgtgggggagcagctcactgcacctcagaagtcaacgttaaaagtcattgtgagcacctagaagtgaagttccacgagacagaaaactgagccacaagatgcccccaaagtaggagtcatgttgaaaactttgaaaaatgtctttgtacaacatctacacagatctttagagaacaggccagacctgtgctgacttaggtactgcctaaaatgtcactatatgaggaaccatttcagcagcatactgcccacgcttctctgagccaaagatgttcctagcactgcctttagccatatcatctttaagtgaaaataagattttatacatattccggctgggacacctcgagcacatgtgacctcaggaaattccttaacttctattcccctagtttccttatctataagatggtgaagattgtggcagaattaaatgagttaatgtgcccgacacataatacaaactactctgcgttagttgtccattagtattatcatccacttatcatatccactcataatttttgcagagaagccaccagcacaaaataaaatcaattacaacacaatttttttcaaaacgtgaacagatactattttataaaaaggttcataggatccccaaattagtattaactcggctcagatttatctaccctaagcacgtggggattcttcccagctcccacgctccttgccaccctaaatgctcaaggggagtcctattgtattagaaatgaacttgctaatcacgactttggacctgatccaagacatgcttttcaggcacagcactggtaaggagatgggtcccctccagaaaatgctgagaaatggtagcaaacaggattccctccttcggtctactcctcactgccttccctctgtgggagatgaagcattgctcccccaatcccatgcacatttgattgctagcctgctggcacaaccctatgatccagtgtgtccagagagatccagatttctccctccgtacgttttctctctctggttggtcctgtctatagctacagatgagcaagaagcatccatggactgcccagggctttcgtttcccatacctctgctgtttgagatctggagaacagaacacatccagtcagtagctcacaccccccatcacattctcagccttcacatgtgaggaaaacagctggtcaaggaaggctgctgaattccatttataagccacttagcaagttatgaagctagaagggtcatttctgtagtcactgtgttattgttacagcatatactgatcacctactggctctaggaagtgagaatgatactttcagttcaaatcttagtgtcaggatttaatatcaaacaggaagaaactctacacctttgctgcttgtcttagccaagcaaatgagggtgtcagagaaactgaccaccctctctaggctgaaatgggttagagcagatctcaacttctggaatttttagttgtggaacctttcctggtaaactattattttaatgtcaatattctgggaggcaggcaaatttaaggcaagagagtacactaaatcataggcacagtggctcacacctgtaatcccaacactttcggaggccgaggcaggcagatcatttgaagtcaggagttcaagaccagcctgggcaacatggtgaaaccccatctcgactaaaaatacaaaaattagctgggtgtggtggtgcatgcctgtaatcccagctacttgggaggcagaggcaggagaatcacttgaacctgggaggcagaggttgcagtgagccaaaatcatgccactgcattctagcctaaacaacagagcgagactcaaaaaaaaaaaaaaaaaaatcatagacacagtgacaatggaaatgtttattgctggtggttgggtctgtcatttcctagaggacatagctggccagcagattttcatttcttttttacaaaataaacaaatgcctactttattatttatacacagaaaattatatagaaacaccacacaaactgcttgaaatacaaatattctttggtttacttatcaaagtaaaaaataacaaaaatcttatcagttaaataaaaaagtgacattctttatcaagccttcttaaacactgaaacgcacgcatttttatgctcatgttctttagcagtatttctccccttttgcccctcattcccctaaattgtttcaatgagttcatctgtagaatgaagattgttacctttcttaatgctacttactttttattatctcaatatcaagaccaatctagacttttttgtctcttacatgtgaaatggatgtaaaaaatggaaaattcaccagcactttttaagataacataaaagaagccctaagcaagcatttcaaggcaatgacacaccattacatttctgagaaatttaagtatcattggtacttaaaaggagaactcaattccagaagcatattcttatactggacattattcataatagctaatatagttcatttccacagtactgatttcagataagccattttttttttcctgagggttgactacctcagacttaaatcctgaatgtcgatgactcaatcttaacaaaacagtcagctgtagacatgaaaattgaattgtttcaaaaggagcaatgatagcaagagaaagttcttggcattttaagaaaagtacatatacatagcaagaaatgaaagtaaatcaaaatacatagctttgtacatgttagaaatatccaatgtgccaccaacacaacaactgccctattaaaaagtcctcaggtctggagacatctgtatttttctttgtataactacatttgcattacccaaccacatatctctcccatggtctgttacccgttaggaagcttttaaccagaatttttggcaatatgcttttcttcaaataaaacaagccttcaaataaatcattatgtctgacaactgaattgggtaaagtctttctgaaatatgtgtaatctttagaaaattcttcttttttccttcataaatcagcagtgctccatcttcaaataaatcatgatcagtcacaatcttaactcatgtgctcatatgttctcttcatccaacattttgttgataccatcacatagtttttgtaagtggggtttaaaattcccaaaaggattatacaaggcagccaaaaattcacaatctgaaaaatgatcaaacacattattaacccgtccatgtgacttggcagtgaggtggcgctgaatgatttggtgcagcatctctctgcattcatttaacagcctggataacacattccggtcaaaggtataatccacctgatggaaactgaccacggtcatagcaagctgatgaactttcttcttaaatttctccatcaatgctagctcatcttgattaaactgattattcctataaagaatggccagcttgatgactgtcttgatgaggttcttgatgatcttctctgcctccttcttgttttgggtgtactccctggtcactctgtagagctcatccagcacctcactacttgtgtcgtctattaaggtggtggcgatggatttggacaccattttacccaagatcttcttttgtgcctgaacggccaggtttttggaattaaagacatctgtggccactgtggttccagctactcaggagactgaggtgggaggatcgcttgagcccaggagttagaggctgcagtgagctatgatctcaccactgcacttcagcctgggtgacacaggaagatcctgttcggaggagtggcgcgacggcgccgggacgctgaagcgcgagctgggctgtttggcggcgccgagttctctgctctctcggtggctcacgggttcccgcggaccttagccaagcgcgggttagagccggcgggagaaaaggaggcagag

SEQ ID NO: 14161 - RNA, 5885 nt, Homo sapiens
  source 1..5885: mol_type = other RNA
gctgggattacaggcatgagccaccgcactcagcctggcagttttaaacgaatgaattcatctgtaagcttttgaatggaaaaaccaaagtagaaagaaacatattgtcttacattattctacaaatcaaaacttttaaaaatcaaattgtctttcttgtattaagaacaaaccgcaagtgcctgatcatctactttatttccacgaggcagaaatacagttatgcagctgatgtcagggaaggcggagaatttcctcagccatccatgaagaaagataaggggccttatccactggctgtctaatcttataaagatctcatgcaaatttggtggacatagggcacaattctctatccttgaagaacattttccaaagcacagatgtttttctcttaattgtgaatgctgactgacttgtccatatcctttctcagtgctcagcagatggtacgatttgggactcgcttgttccctataacgtggggctgatgttctttgctacgtggaaaacacatctttggtgagacagaaatgaatcaatattacacaaaaatgtttccatttctggaatttccctgagataaaaatatctttctggctttgggtatacataagtgaccgtgcagacacttagtaaaagagaaaacagattttcaatacttcgtggtgatggtgactatacgggattataagtagttaaaggttttcctgttgcatcattttggaaacaaaaagctgactcattttctggttaatgcttcaatattttcattagggagtttctataaagtttttatctgaatcacagaaagtacaattatttcagaggtaggataaaattttttctgtcataaacagcactgtgtactaaaacctgctatgagtttaacaaatcacctagaagcctaatgctcaagaatgcaatatatcaagtaaaacactgaaaagttcaactagtttagataatgcaagtatggaaatgcaagattgactaaaacttttaaatattatcactcttattaacatgctaatttaattcattttactggagtattttaatttcctggcaattgaatagcactttttactacaaatatttcatcatttggataaacatattcttttatttaccatttgtcaggttttgtatgctaaattgcaactgcttatatacactcatcaagtatctcaaggataaattaaaattcttagtaaaaatccaactgaccggtacagaccacaaaaagtactattttaagcctttgggggcttaaaaattgtgtgtgtgtgtgtgtgtgtgtgtgtattcacatggtgggagaaaaagaactttccagataattgtgaatggcatactattatataagagtttaaaacgcaatatttctgtacgatcaaagttcttaactcatgctttttttttttttttttttttttgagacggggtttcgttcttgttgcccaggctgcagtgcagtggtacaatctcagctcactgcaacctctgcctcccaggttccagcgattctcctgccttagcctcccaagtagctgggattacaggtgcctgccaccacatctggctaatcttgtgtatttttagtagcagtggggtttcaccacgttggccaggctggtctcgaactcctcacctcaagtgatcctcccacctccgcctcccaaagttctgggcttacaagcataagccaccgcacccaccccatgctttactcttaaactaattttgagttgtatatgaaaggcctaataatcagaaaaaggctatttcttaacttaacttgctcaaatattttgagcctccaaatctggaaaataatgttgaagtttgaaactgatgccgtgcctactctagggagcacagtactgaactgctgcttccttgcttctcttggtgaatgcacattgagtgccttgtcatgctctgaacccaccactgctagggacagctgtgggggagcagctcactgcacctcagaagtcaacgttaaaagtcattgtgagcacctagaagtgaagttccacgagacagaaaactgagccacaagatgcccccaaagtaggagtcatgttgaaaactttgaaaaatgtctttgtacaacatctacacagatctttagagaacaggccagacctgtgctgacttaggtactgcctaaaatgtcactatatgaggaaccatttcagcagcatactgcccacgcttctctgagccaaagatgttcctagcactgcctttagccatatcatctttaagtgaaaataagattttatacatattccggctgggacacctcgagcacatgtgacctcaggaaattccttaacttctattcccctagtttccttatctataagatggtgaagattgtggcagaattaaatgagttaatgtgcccgacacataatacaaactactctgcgttagttgtccattagtattatcatccacttatcatatccactcataatttttgcagagaagccaccagcacaaaataaaatcaattacaacacaatttttttcaaaacgtgaacagatactattttataaaaaggttcataggatccccaaattagtattaactcggctcagatttatctaccctaagcacgtggggattcttcccagctcccacgctccttgccaccctaaatgctcaaggggagtcctattgtattagaaatgaacttgctaatcacgactttggacctgatccaagacatgcttttcaggcacagcactggtaaggagatgggtcccctccagaaaatgctgagaaatggtagcaaacaggattccctccttcggtctactcctcactgccttccctctgtgggagatgaagcattgctcccccaatcccatgcacatttgattgctagcctgctggcacaaccctatgatccagtgtgtccagagagatccagatttctccctccgtacgttttctctctctggttggtcctgtctatagctacagatgagcaagaagcatccatggactgcccagggctttcgtttcccatacctctgctgtttgagatctggagaacagaacacatccagtcagtagctcacaccccccatcacattctcagccttcacatgtgaggaaaacagctggtcaaggaaggctgctgaattccatttataagccacttagcaagttatgaagctagaagggtcatttctgtagtcactgtgttattgttacagcatatactgatcacctactggctctaggaagtgagaatgatactttcagttcaaatcttagtgtcaggatttaatatcaaacaggaagaaactctacacctttgctgcttgtcttagccaagcaaatgagggtgtcagagaaactgaccaccctctctaggctgaaatgggttagagcagatctcaacttctggaatttttagttgtggaacctttcctggtaaactattattttaatgtcaatattctgggaggcaggcaaatttaaggcaagagagtacactaaatcataggcacagtggctcacacctgtaatcccaacactttcggaggccgaggcaggcagatcatttgaagtcaggagttcaagaccagcctgggcaacatggtgaaaccccatctcgactaaaaatacaaaaattagctgggtgtggtggtgcatgcctgtaatcccagctacttgggaggcagaggcaggagaatcacttgaacctgggaggcagaggttgcagtgagccaaaatcatgccactgcattctagcctaaacaacagagcgagactcaaaaaaaaaaaaaaaaaaatcatagacacagtgacaatggaaatgtttattgctggtggttgggtctgtcatttcctagaggacatagctggccagcagattttcatttcttttttacaaaataaacaaatgcctactttattatttatacacagaaaattatatagaaacaccacacaaactgcttgaaatacaaatattctttggtttacttatcaaagtaaaaaataacaaaaatcttatcagttaaataaaaaagtgacattctttatcaagccttcttaaacactgaaacgcacgcatttttatgctcatgttctttagcagtatttctccccttttgcccctcattcccctaaattgtttcaatgagttcatctgtagaatgaagattgttacctttcttaatgctacttactttttattatctcaatatcaagaccaatctagacttttttgtctcttacatgtgaaatggatgtaaaaaatggaaaattcaccagcactttttaagataacataaaagaagccctaagcaagcatttcaaggcaatgacacaccattacatttctgagaaatttaagtatcattggtacttaaaaggagaactcaattccagaagcatattcttatactggacattattcataatagctaatatagttcatttccacagtactgatttcagataagccattttttttttcctgagggttgactacctcagacttaaatcctgaatgtcgatgactcaatcttaacaaaacagtcagctgtagacatgaaaattgaattgtttcaaaaggagcaatgatagcaagagaaagttcttggcattttaagaaaagtacatatacatagcaagaaatgaaagtaaatcaaaatacatagctttgtacatgttagaaatatccaatgtgccaccaacacaacaactgccctattaaaaagtcctcaggtctggagacatctgtatttttctttgtataactacatttgcattacccaaccacatatctctcccatggtctgttacccgttaggaagcttttaaccagaatttttggcaatatgcttttcttcaaataaaacaagccttcaaataaatcattatgtctgacaactgaattgggtaaagtctttctgaaatatgtgtaatctttagaaaattcttcttttttccttcataaatcagcagtgctccatcttcaaataaatcatgatcagtcacaatcttaactcatgtgctcatatgttctcttcatccaacattttgttgataccatcacatagtttttgtaagtggggtttaaaattcccaaaaggattatacaaggcagccaaaaattcacaatctgaaaaatgatcaaacacattattaacccgtccatgtgacttggcagtgaggtggcgctgaatgatttggtgcagcatctctctgcattcatttaacagcctggataacacattccggtcaaaggtataatccacctgatggaaactgaccacggtcatagcaagctgatgaactttcttcttaaatttctccatcaatgctagctcatcttgattaaactgattattcctataaagaatggccagcttgatgactgtcttgatgaggttcttgatgatcttctctgcctccttcttgttttgggtgtactccctggtcactctgtagagctcatccagcacctcactacttgtgtcgtctattaaggtggtggcgatggatttggacaccattttacccaagatcttcttttgtgcctgaacggccaggtttttggaattaaagacatctgtggccactgtggttccagctactcaggagactgaggtgggaggatcgcttgagcccaggagttagaggctgcagtgagctatgatctcaccactgcacttcagcctgggtgacacaggaagatctcggaggagtggcgcgacggcgccgggacgctgaagcgcgagctgggctgtttggcggcgccgagttctctgctctctcggtggctcacgggttcccgcggaccttagccaagcgcgggttagagccggcgggagaaaaggaggcagag

SEQ ID NO: 14162 - RNA, 5721 nt, Homo sapiens
  source 1..5721: mol_type = other RNA
gctgggattacaggcatgagccaccgcactcagcctggcagttttaaacgaatgaattcatctgtaagcttttgaatggaaaaaccaaagtagaaagaaacatattgtcttacattattctacaaatcaaaacttttaaaaatcaaattgtctttcttgtattaagaacaaaccgcaagtgcctgatcatctactttatttccacgaggcagaaatacagttatgcagctgatgtcagggaaggcggagaatttcctcagccatccatgaagaaagataaggggccttatccactggctgtctaatcttataaagatctcatgcaaatttggtggacatagggcacaattctctatccttgaagaacattttccaaagcacagatgtttttctcttaattgtgaatgctgactgacttgtccatatcctttctcagtgctcagcagatggtacgatttgggactcgcttgttccctataacgtggggctgatgttctttgctacgtggaaaacacatctttggtgagacagaaatgaatcaatattacacaaaaatgtttccatttctggaatttccctgagataaaaatatctttctggctttgggtatacataagtgaccgtgcagacacttagtaaaagagaaaacagattttcaatacttcgtggtgatggtgactatacgggattataagtagttaaaggttttcctgttgcatcattttggaaacaaaaagctgactcattttctggttaatgcttcaatattttcattagggagtttctataaagtttttatctgaatcacagaaagtacaattatttcagaggtaggataaaattttttctgtcataaacagcactgtgtactaaaacctgctatgagtttaacaaatcacctagaagcctaatgctcaagaatgcaatatatcaagtaaaacactgaaaagttcaactagtttagataatgcaagtatggaaatgcaagattgactaaaacttttaaatattatcactcttattaacatgctaatttaattcattttactggagtattttaatttcctggcaattgaatagcactttttactacaaatatttcatcatttggataaacatattcttttatttaccatttgtcaggttttgtatgctaaattgcaactgcttatatacactcatcaagtatctcaaggataaattaaaattcttagtaaaaatccaactgaccggtacagaccacaaaaagtactattttaagcctttgggggcttaaaaattgtgtgtgtgtgtgtgtgtgtgtgtgtattcacatggtgggagaaaaagaactttccagataattgtgaatggcatactattatataagagtttaaaacgcaatatttctgtacgatcaaagttcttaactcatgctttttttttttttttttttttttgagacggggtttcgttcttgttgcccaggctgcagtgcagtggtacaatctcagctcactgcaacctctgcctcccaggttccagcgattctcctgccttagcctcccaagtagctgggattacaggtgcctgccaccacatctggctaatcttgtgtatttttagtagcagtggggtttcaccacgttggccaggctggtctcgaactcctcacctcaagtgatcctcccacctccgcctcccaaagttctgggcttacaagcataagccaccgcacccaccccatgctttactcttaaactaattttgagttgtatatgaaaggcctaataatcagaaaaaggctatttcttaacttaacttgctcaaatattttgagcctccaaatctggaaaataatgttgaagtttgaaactgatgccgtgcctactctagggagcacagtactgaactgctgcttccttgcttctcttggtgaatgcacattgagtgccttgtcatgctctgaacccaccactgctagggacagctgtgggggagcagctcactgcacctcagaagtcaacgttaaaagtcattgtgagcacctagaagtgaagttccacgagacagaaaactgagccacaagatgcccccaaagtaggagtcatgttgaaaactttgaaaaatgtctttgtacaacatctacacagatctttagagaacaggccagacctgtgctgacttaggtactgcctaaaatgtcactatatgaggaaccatttcagcagcatactgcccacgcttctctgagccaaagatgttcctagcactgcctttagccatatcatctttaagtgaaaataagattttatacatattccggctgggacacctcgagcacatgtgacctcaggaaattccttaacttctattcccctagtttccttatctataagatggtgaagattgtggcagaattaaatgagttaatgtgcccgacacataatacaaactactctgcgttagttgtccattagtattatcatccacttatcatatccactcataatttttgcagagaagccaccagcacaaaataaaatcaattacaacacaatttttttcaaaacgtgaacagatactattttataaaaaggttcataggatccccaaattagtattaactcggctcagatttatctaccctaagcacgtggggattcttcccagctcccacgctccttgccaccctaaatgctcaaggggagtcctattgtattagaaatgaacttgctaatcacgactttggacctgatccaagacatgcttttcaggcacagcactggtaaggagatgggtcccctccagaaaatgctgagaaatggtagcaaacaggattccctccttcggtctactcctcactgccttccctctgtgggagatgaagcattgctcccccaatcccatgcacatttgattgctagcctgctggcacaaccctatgatccagtgtgtccagagagatccagatttctccctccgtacgttttctctctctggttggtcctgtctatagctacagatgagcaagaagcatccatggactgcccagggctttcgtttcccatacctctgctgtttgagatctggagaacagaacacatccagtcagtagctcacaccccccatcacattctcagccttcacatgtgaggaaaacagctggtcaaggaaggctgctgaattccatttataagccacttagcaagttatgaagctagaagggtcatttctgtagtcactgtgttattgttacagcatatactgatcacctactggctctaggaagtgagaatgatactttcagttcaaatcttagtgtcaggatttaatatcaaacaggaagaaactctacacctttgctgcttgtcttagccaagcaaatgagggtgtcagagaaactgaccaccctctctaggctgaaatgggttagagcagatctcaacttctggaatttttagttgtggaacctttcctggtaaactattattttaatgtcaatattctgggaggcaggcaaatttaaggcaagagagtacactaaatcataggcacagtggctcacacctgtaatcccaacactttcggaggccgaggcaggcagatcatttgaagtcaggagttcaagaccagcctgggcaacatggtgaaaccccatctcgactaaaaatacaaaaattagctgggtgtggtggtgcatgcctgtaatcccagctacttgggaggcagaggcaggagaatcacttgaacctgggaggcagaggttgcagtgagccaaaatcatgccactgcattctagcctaaacaacagagcgagactcaaaaaaaaaaaaaaaaaaatcatagacacagtgacaatggaaatgtttattgctggtggttgggtctgtcatttcctagaggacatagctggccagcagattttcatttcttttttacaaaataaacaaatgcctactttattatttatacacagaaaattatatagaaacaccacacaaactgcttgaaatacaaatattctttggtttacttatcaaagtaaaaaataacaaaaatcttatcagttaaataaaaaagtgacattctttatcaagccttcttaaacactgaaacgcacgcatttttatgctcatgttctttagcagtatttctccccttttgcccctcattcccctaaattgtttcaatgagttcatctgtagaatgaagattgttacctttcttaatgctacttactttttattatctcaatatcaagaccaatctagacttttttgtctcttacatgtgaaatggatgtaaaaaatggaaaattcaccagcactttttaagataacataaaagaagccctaagcaagcatttcaaggcaatgacacaccattacatttctgagaaatttaagtatcattggtacttaaaaggagaactcaattccagaagcatattcttatactggacattattcataatagctaatatagttcatttccacagtactgatttcagataagccattttttttttcctgagggttgactacctcagacttaaatcctgaatgtcgatgactcaatcttaacaaaacagtcagctgtagacatgaaaattgaattgtttcaaaaggagcaatgatagcaagagaaagttcttggcattttaagaaaagtacatatacatagcaagaaatgaaagtaaatcaaaatacatagctttgtacatgttagaaatatccaatgtgccaccaacacaacaactgccctattaaaaagtcctcaggtctggagacatctgtatttttctttgtataactacatttgcattacccaaccacatatctctcccatggtctgttacccgttaggaagcttttaaccagaatttttggcaatatgcttttcttcaaataaaacaagccttcaaataaatcattatgtctgacaactgaattgggtaaagtctttctgaaatatgtgtaatctttagaaaattcttcttttttccttcataaatcagcagtgctccatcttcaaataaatcatgatcagtcacaatcttaactcatgtgctcatatgttctcttcatccaacattttgttgataccatcacatagtttttgtaagtggggtttaaaattcccaaaaggattatacaaggcagccaaaaattcacaatctgaaaaatgatcaaacacattattaacccgtccatgtgacttggcagtgaggtggcgctgaatgatttggtgcagcatctctctgcattcatttaacagcctggataacacattccggtcaaaggtataatccacctgatggaaactgaccacggtcatagcaagctgatgaactttcttcttaaatttctccatcaatgctagctcatcttgattaaactgattattcctataaagaatggccagcttgatgactgtcttgatgaggttcttgatgatcttctctgcctccttcttgttttgggtgtactccctggtcactctgtagagctcatccagcacctcactacttgtgtcgtctattaaggtggtggcgatggatttggacaccattttacccaagatcttcttttgtgcctgaacggccaggtttttggaattaaagacatctgtggccacttccttggattcttctgcttcggagtgcataatgtcaggataaccagctgcaggggcgattaccgctcacatgtactcggacgagccgcaagttcgctctgc

SEQ ID NO: 14163 - RNA, 6337 nt, Homo sapiens
  source 1..6337: mol_type = other RNA
gctgggattacaggcatgagccaccgcactcagcctggcagttttaaacgaatgaattcatctgtaagcttttgaatggaaaaaccaaagtagaaagaaacatattgtcttacattattctacaaatcaaaacttttaaaaatcaaattgtctttcttgtattaagaacaaaccgcaagtgcctgatcatctactttatttccacgaggcagaaatacagttatgcagctgatgtcagggaaggcggagaatttcctcagccatccatgaagaaagataaggggccttatccactggctgtctaatcttataaagatctcatgcaaatttggtggacatagggcacaattctctatccttgaagaacattttccaaagcacagatgtttttctcttaattgtgaatgctgactgacttgtccatatcctttctcagtgctcagcagatggtacgatttgggactcgcttgttccctataacgtggggctgatgttctttgctacgtggaaaacacatctttggtgagacagaaatgaatcaatattacacaaaaatgtttccatttctggaatttccctgagataaaaatatctttctggctttgggtatacataagtgaccgtgcagacacttagtaaaagagaaaacagattttcaatacttcgtggtgatggtgactatacgggattataagtagttaaaggttttcctgttgcatcattttggaaacaaaaagctgactcattttctggttaatgcttcaatattttcattagggagtttctataaagtttttatctgaatcacagaaagtacaattatttcagaggtaggataaaattttttctgtcataaacagcactgtgtactaaaacctgctatgagtttaacaaatcacctagaagcctaatgctcaagaatgcaatatatcaagtaaaacactgaaaagttcaactagtttagataatgcaagtatggaaatgcaagattgactaaaacttttaaatattatcactcttattaacatgctaatttaattcattttactggagtattttaatttcctggcaattgaatagcactttttactacaaatatttcatcatttggataaacatattcttttatttaccatttgtcaggttttgtatgctaaattgcaactgcttatatacactcatcaagtatctcaaggataaattaaaattcttagtaaaaatccaactgaccggtacagaccacaaaaagtactattttaagcctttgggggcttaaaaattgtgtgtgtgtgtgtgtgtgtgtgtgtattcacatggtgggagaaaaagaactttccagataattgtgaatggcatactattatataagagtttaaaacgcaatatttctgtacgatcaaagttcttaactcatgctttttttttttttttttttttttgagacggggtttcgttcttgttgcccaggctgcagtgcagtggtacaatctcagctcactgcaacctctgcctcccaggttccagcgattctcctgccttagcctcccaagtagctgggattacaggtgcctgccaccacatctggctaatcttgtgtatttttagtagcagtggggtttcaccacgttggccaggctggtctcgaactcctcacctcaagtgatcctcccacctccgcctcccaaagttctgggcttacaagcataagccaccgcacccaccccatgctttactcttaaactaattttgagttgtatatgaaaggcctaataatcagaaaaaggctatttcttaacttaacttgctcaaatattttgagcctccaaatctggaaaataatgttgaagtttgaaactgatgccgtgcctactctagggagcacagtactgaactgctgcttccttgcttctcttggtgaatgcacattgagtgccttgtcatgctctgaacccaccactgctagggacagctgtgggggagcagctcactgcacctcagaagtcaacgttaaaagtcattgtgagcacctagaagtgaagttccacgagacagaaaactgagccacaagatgcccccaaagtaggagtcatgttgaaaactttgaaaaatgtctttgtacaacatctacacagatctttagagaacaggccagacctgtgctgacttaggtactgcctaaaatgtcactatatgaggaaccatttcagcagcatactgcccacgcttctctgagccaaagatgttcctagcactgcctttagccatatcatctttaagtgaaaataagattttatacatattccggctgggacacctcgagcacatgtgacctcaggaaattccttaacttctattcccctagtttccttatctataagatggtgaagattgtggcagaattaaatgagttaatgtgcccgacacataatacaaactactctgcgttagttgtccattagtattatcatccacttatcatatccactcataatttttgcagagaagccaccagcacaaaataaaatcaattacaacacaatttttttcaaaacgtgaacagatactattttataaaaaggttcataggatccccaaattagtattaactcggctcagatttatctaccctaagcacgtggggattcttcccagctcccacgctccttgccaccctaaatgctcaaggggagtcctattgtattagaaatgaacttgctaatcacgactttggacctgatccaagacatgcttttcaggcacagcactggtaaggagatgggtcccctccagaaaatgctgagaaatggtagcaaacaggattccctccttcggtctactcctcactgccttccctctgtgggagatgaagcattgctcccccaatcccatgcacatttgattgctagcctgctggcacaaccctatgatccagtgtgtccagagagatccagatttctccctccgtacgttttctctctctggttggtcctgtctatagctacagatgagcaagaagcatccatggactgcccagggctttcgtttcccatacctctgctgtttgagatctggagaacagaacacatccagtcagtagctcacaccccccatcacattctcagccttcacatgtgaggaaaacagctggtcaaggaaggctgctgaattccatttataagccacttagcaagttatgaagctagaagggtcatttctgtagtcactgtgttattgttacagcatatactgatcacctactggctctaggaagtgagaatgatactttcagttcaaatcttagtgtcaggatttaatatcaaacaggaagaaactctacacctttgctgcttgtcttagccaagcaaatgagggtgtcagagaaactgaccaccctctctaggctgaaatgggttagagcagatctcaacttctggaatttttagttgtggaacctttcctggtaaactattattttaatgtcaatattctgggaggcaggcaaatttaaggcaagagagtacactaaatcataggcacagtggctcacacctgtaatcccaacactttcggaggccgaggcaggcagatcatttgaagtcaggagttcaagaccagcctgggcaacatggtgaaaccccatctcgactaaaaatacaaaaattagctgggtgtggtggtgcatgcctgtaatcccagctacttgggaggcagaggcaggagaatcacttgaacctgggaggcagaggttgcagtgagccaaaatcatgccactgcattctagcctaaacaacagagcgagactcaaaaaaaaaaaaaaaaaaatcatagacacagtgacaatggaaatgtttattgctggtggttgggtctgtcatttcctagaggacatagctggccagcagattttcatttcttttttacaaaataaacaaatgcctactttattatttatacacagaaaattatatagaaacaccacacaaactgcttgaaatacaaatattctttggtttacttatcaaagtaaaaaataacaaaaatcttatcagttaaataaaaaagtgacattctttatcaagccttcttaaacactgaaacgcacgcatttttatgctcatgttctttagcagtatttctccccttttgcccctcattcccctaaattgtttcaatgagttcatctgtagaatgaagattgttacctttcttaatgctacttactttttattatctcaatatcaagaccaatctagacttttttgtctcttacatgtgaaatggatgtaaaaaatggaaaattcaccagcactttttaagataacataaaagaagccctaagcaagcatttcaaggcaatgacacaccattacatttctgagaaatttaagtatcattggtacttaaaaggagaactcaattccagaagcatattcttatactggacattattcataatagctaatatagttcatttccacagtactgatttcagataagccattttttttttcctgagggttgactacctcagacttaaatcctgaatgtcgatgactcaatcttaacaaaacagtcagctgtagacatgaaaattgaattgtttcaaaaggagcaatgatagcaagagaaagttcttggcattttaagaaaagtacatatacatagcaagaaatgaaagtaaatcaaaatacatagctttgtacatgttagaaatatccaatgtgccaccaacacaacaactgccctattaaaaagtcctcaggtctggagacatctgtatttttctttgtataactacatttgcattacccaaccacatatctctcccatggtctgttacccgttaggaagcttttaaccagaatttttggcaatatgcttttcttcaaataaaacaagccttcaaataaatcattatgtctgacaactgaattgggtaaagtctttctgaaatatgtgtaatctttagaaaattcttcttttttccttcataaatcagcagtgctccatcttcaaataaatcatgatcagtcacaatcttaactcatgtgctcatatgttctcttcatccaacattttgttgataccatcacatagtttttgtaagtggggtttaaaattcccaaaaggattatacaaggcagccaaaaattcacaatctgaaaaatgatcaaacacattattaacccgtccatgtgacttggcagtgaggtggcgctgaatgatttggtgcagcatctctctgcattcatttaacagcctggataacacattccggtcaaaggtataatccacctgatggaaactgaccacggtcatagcaagctgatgaactttcttcttaaatttctccatcaatgctagctcatcttgattaaactgattattcctataaagaatggccagcttgatgactgtcttgatgaggttcttgatgatcttctctgcctccttcttgttttgggtgtactccctggtcactctgtagagctcatccagcacctcactacttgtgtcgtctattaaggtggtggcgatggatttggacaccattttacccaagatcttcttttgtgcctgaacggccaggtttttggaattaaagacatctgtggccacttccttggattcttctgcttcggagtgcataatgtcaggataaccagctgcaggggcgattaccgctcacatgtactcggacgagccgcaagttcgctctttgcacagcaaaagcagacggggctgcttactcattcagtatagccccgggcgagcactggtactccaagcacagcccgggcactcattgctgcagttactccaaagggccttcctcagggggagagcacggttccctcccggctaccagcaaaaactggggatgaattccttcaaaatgccaaaggggaggttttcaggatttgaaatgctgatagaataaagaagccggacagccttcacaacagatctcaattctgcccccgggtctggcccacaggcccctacaaattggctgagaggaagtccccttagctctgtggagccttggttttcccttctgcaaagcggggacaagagctgccactgataggcctgtcttacggaggtattttgtagaacacttgttttatcgccagtctgaggcaaaaagtcctcaaataacatatctgaaagatccgcttggaaattatgagaaaaaaatatactcttttgacaaatttattttccagttcgtttctttttcttcgtttccgattttatataggcaaaaaccaatagaaacactatggcaaatttagtgaaaagaacgtacaaaagacatggatttaaggagtct

SEQ ID NO: 14164 - RNA, 5767 nt, Homo sapiens
  source 1..5767: mol_type = other RNA
gctgggattacaggcatgagccaccgcactcagcctggcagttttaaacgaatgaattcatctgtaagcttttgaatggaaaaaccaaagtagaaagaaacatattgtcttacattattctacaaatcaaaacttttaaaaatcaaattgtctttcttgtattaagaacaaaccgcaagtgcctgatcatctactttatttccacgaggcagaaatacagttatgcagctgatgtcagggaaggcggagaatttcctcagccatccatgaagaaagataaggggccttatccactggctgtctaatcttataaagatctcatgcaaatttggtggacatagggcacaattctctatccttgaagaacattttccaaagcacagatgtttttctcttaattgtgaatgctgactgacttgtccatatcctttctcagtgctcagcagatggtacgatttgggactcgcttgttccctataacgtggggctgatgttctttgctacgtggaaaacacatctttggtgagacagaaatgaatcaatattacacaaaaatgtttccatttctggaatttccctgagataaaaatatctttctggctttgggtatacataagtgaccgtgcagacacttagtaaaagagaaaacagattttcaatacttcgtggtgatggtgactatacgggattataagtagttaaaggttttcctgttgcatcattttggaaacaaaaagctgactcattttctggttaatgcttcaatattttcattagggagtttctataaagtttttatctgaatcacagaaagtacaattatttcagaggtaggataaaattttttctgtcataaacagcactgtgtactaaaacctgctatgagtttaacaaatcacctagaagcctaatgctcaagaatgcaatatatcaagtaaaacactgaaaagttcaactagtttagataatgcaagtatggaaatgcaagattgactaaaacttttaaatattatcactcttattaacatgctaatttaattcattttactggagtattttaatttcctggcaattgaatagcactttttactacaaatatttcatcatttggataaacatattcttttatttaccatttgtcaggttttgtatgctaaattgcaactgcttatatacactcatcaagtatctcaaggataaattaaaattcttagtaaaaatccaactgaccggtacagaccacaaaaagtactattttaagcctttgggggcttaaaaattgtgtgtgtgtgtgtgtgtgtgtgtgtattcacatggtgggagaaaaagaactttccagataattgtgaatggcatactattatataagagtttaaaacgcaatatttctgtacgatcaaagttcttaactcatgctttttttttttttttttttttttgagacggggtttcgttcttgttgcccaggctgcagtgcagtggtacaatctcagctcactgcaacctctgcctcccaggttccagcgattctcctgccttagcctcccaagtagctgggattacaggtgcctgccaccacatctggctaatcttgtgtatttttagtagcagtggggtttcaccacgttggccaggctggtctcgaactcctcacctcaagtgatcctcccacctccgcctcccaaagttctgggcttacaagcataagccaccgcacccaccccatgctttactcttaaactaattttgagttgtatatgaaaggcctaataatcagaaaaaggctatttcttaacttaacttgctcaaatattttgagcctccaaatctggaaaataatgttgaagtttgaaactgatgccgtgcctactctagggagcacagtactgaactgctgcttccttgcttctcttggtgaatgcacattgagtgccttgtcatgctctgaacccaccactgctagggacagctgtgggggagcagctcactgcacctcagaagtcaacgttaaaagtcattgtgagcacctagaagtgaagttccacgagacagaaaactgagccacaagatgcccccaaagtaggagtcatgttgaaaactttgaaaaatgtctttgtacaacatctacacagatctttagagaacaggccagacctgtgctgacttaggtactgcctaaaatgtcactatatgaggaaccatttcagcagcatactgcccacgcttctctgagccaaagatgttcctagcactgcctttagccatatcatctttaagtgaaaataagattttatacatattccggctgggacacctcgagcacatgtgacctcaggaaattccttaacttctattcccctagtttccttatctataagatggtgaagattgtggcagaattaaatgagttaatgtgcccgacacataatacaaactactctgcgttagttgtccattagtattatcatccacttatcatatccactcataatttttgcagagaagccaccagcacaaaataaaatcaattacaacacaatttttttcaaaacgtgaacagatactattttataaaaaggttcataggatccccaaattagtattaactcggctcagatttatctaccctaagcacgtggggattcttcccagctcccacgctccttgccaccctaaatgctcaaggggagtcctattgtattagaaatgaacttgctaatcacgactttggacctgatccaagacatgcttttcaggcacagcactggtaaggagatgggtcccctccagaaaatgctgagaaatggtagcaaacaggattccctccttcggtctactcctcactgccttccctctgtgggagatgaagcattgctcccccaatcccatgcacatttgattgctagcctgctggcacaaccctatgatccagtgtgtccagagagatccagatttctccctccgtacgttttctctctctggttggtcctgtctatagctacagatgagcaagaagcatccatggactgcccagggctttcgtttcccatacctctgctgtttgagatctggagaacagaacacatccagtcagtagctcacaccccccatcacattctcagccttcacatgtgaggaaaacagctggtcaaggaaggctgctgaattccatttataagccacttagcaagttatgaagctagaagggtcatttctgtagtcactgtgttattgttacagcatatactgatcacctactggctctaggaagtgagaatgatactttcagttcaaatcttagtgtcaggatttaatatcaaacaggaagaaactctacacctttgctgcttgtcttagccaagcaaatgagggtgtcagagaaactgaccaccctctctaggctgaaatgggttagagcagatctcaacttctggaatttttagttgtggaacctttcctggtaaactattattttaatgtcaatattctgggaggcaggcaaatttaaggcaagagagtacactaaatcataggcacagtggctcacacctgtaatcccaacactttcggaggccgaggcaggcagatcatttgaagtcaggagttcaagaccagcctgggcaacatggtgaaaccccatctcgactaaaaatacaaaaattagctgggtgtggtggtgcatgcctgtaatcccagctacttgggaggcagaggcaggagaatcacttgaacctgggaggcagaggttgcagtgagccaaaatcatgccactgcattctagcctaaacaacagagcgagactcaaaaaaaaaaaaaaaaaaatcatagacacagtgacaatggaaatgtttattgctggtggttgggtctgtcatttcctagaggacatagctggccagcagattttcatttcttttttacaaaataaacaaatgcctactttattatttatacacagaaaattatatagaaacaccacacaaactgcttgaaatacaaatattctttggtttacttatcaaagtaaaaaataacaaaaatcttatcagttaaataaaaaagtgacattctttatcaagccttcttaaacactgaaacgcacgcatttttatgctcatgttctttagcagtatttctccccttttgcccctcattcccctaaattgtttcaatgagttcatctgtagaatgaagattgttacctttcttaatgctacttactttttattatctcaatatcaagaccaatctagacttttttgtctcttacatgtgaaatggatgtaaaaaatggaaaattcaccagcactttttaagataacataaaagaagccctaagcaagcatttcaaggcaatgacacaccattacatttctgagaaatttaagtatcattggtacttaaaaggagaactcaattccagaagcatattcttatactggacattattcataatagctaatatagttcatttccacagtactgatttcagataagccattttttttttcctgagggttgactacctcagacttaaatcctgaatgtcgatgactcaatcttaacaaaacagtcagctgtagacatgaaaattgaattgtttcaaaaggagcaatgatagcaagagaaagttcttggcattttaagaaaagtacatatacatagcaagaaatgaaagtaaatcaaaatacatagctttgtacatgttagaaatatccaatgtgccaccaacacaacaactgccctattaaaaagtcctcaggtctggagacatctgtatttttctttgtataactacatttgcattacccaaccacatatctctcccatggtctgttacccgttaggaagcttttaaccagaatttttggcaatatgcttttcttcaaataaaacaagccttcaaataaatcattatgtctgacaactgaattgggtaaagtctttctgaaatatgtgtaatctttagaaaattcttcttttttccttcataaatcagcagtgctccatcttcaaataaatcatgatcagtcacaatcttaactcatgtgctcatatgttctcttcatccaacattttgttgataccatcacatagtttttgtaagtggggtttaaaattcccaaaaggattatacaaggcagccaaaaattcacaatctgaaaaatgatcaaacacattattaacccgtccatgtgacttggcagtgaggtggcgctgaatgatttggtgcagcatctctctgcattcatttaacagcctggataacacattccggtcaaaggtataatccacctgatggaaactgaccacggtcatagcaagctgatgaactttcttcttaaatttctccatcaatgctagctcatcttgattaaactgattattcctataaagaatggccagcttgatgactgtcttgatgaggttcttgatgatcttctctgcctccttcttgttttgggtgtactccctggtcactctgtagagctcatccagcacctcactacttgtgtcgtctattaaggtggtggcgatggatttggacaccattttacccaagatcttcttttgtgcctgaacggccaggtttttggaattaaagacatctgtggccatcggaggagtggcgcgacggcgccgggacgctgaagcgcgagctgggctgtttggcggcgccgagttctctgctctctcggtggctcacgggttcccgcggaccttagccaagcgcgggttagagccggcgggagaaaaggaggcagag

SEQ ID NO: 14165 - RNA, 1679 nt, Homo sapiens
  source 1..1679: mol_type = other RNA
gctgggattacaggcatgagccaccgcactcggcctctgaagagattatccaagtcaatatcttcttttcctttgattttcaaacactttgcctgctgtacaagtctgggctgactgttcaccttttcatgttttccattgaagttcaaactacagaggctttttgattttgaatgtgaagagtctgattccaaatttgcctgtgtttgttctctcaaacgatcgtgaagtgttgcctcctttttcaagttcatgtctgaatacgggcagccaaaagcactgtgatgtcccgaataacgtggaccacggatatggcctattcctcggcacccgggagtaggacagacagcttgacctggaaggatcttcaggtcattcgttcgctgtggcacttccagtggatgccctgtgacatcacaccatccgatcgggtggatatcagggctgtctgcctccacccagtagtcatacttatggtcccaaccatcaaaatgaacctttactctttggtcatcaacatctacaatcgtagcaacacgaattaacctggggttccgtttatccacaacttcaagtttcatatttggcagaaaaccatgaggcaacctcattttaaaaactttggcaggaactgcattggtttgagtagcttccaggtattctgtccaggaaaaattttctggattgggataaccttggggtgctatcagagttcttccattctcctgacaccaaccaactggctggacataagggctattaacatcgcaccagtaatcgtaactatcatcccagttgtcaaaatgcactagtaagcgatcttcaacaatatctgctatggtcgccacacacaccaaggaagggttcttcctgtccacggcctccagcttcattccaacctgaaattctttagacattggcccattaggacttctgtttctgaataatttctttggagcattttgcaatttgcaggccttcaagtaatccatccaaacaaatttatcttttctataacccttagggatgtgcagttcatgtttggtcttttcacaccatcctactggatgaatgtcaggggaaccagcattggtccaaaaatcatagcaacttaaataaccatcaaaatgaagtcttagacggtaaccacaaacctccgctacagaaagcacacagaataccgatggatgtcggggatcaatgccttctaatctcattccaatctgaaaaccattttcatgctctggaaaggactgatccttggaaaacagctcaacaggtgctgcgacagccttctgttctttcaagtaccactcccaagaccatgctccctgtgcagccgctgaagggacgtgactcaaaggggttgtgctatccttgggcttcttttcctcttcagcttgctccaagcgtccgtcctgatccaaacgctctttggaatccatattaagcttccttttcctgttgggctgtttcattgccacccccgcactccttggcagtggttttatggtctgacacgtattcttggtaagaggtcttagtcatacaaggcatagcatagcaatccccagcggagcggcgcctgcccgcaacgccgaccgagctacaggcggggggcgagtcggagcgcgaggttccgccagcccaggctgcggcgccgctgccccgcggtgccc

SEQ ID NO: 14166 - RNA, 4525 nt, Homo sapiens
  source 1..4525: mol_type = other RNA
gctgggattacaggcatgagccaccgcagccagccctgtagcaaacatttttatgtattaagagaatccttttatagacaaagtcttaatctttgtaatgtaacccaactgtgatttcttagcagtgaatcttacatgtggaagagatcactagagttcattcttcatattttcttctttctgagagcagagtttgatttcattctccaggctcccttgctgtcaggtgaggctatgtgaccaagggctggccaatgaaagtggtcataagtagttcacaccacttccaggactgtcccataaagacacacccctcccttccccataattcttaatttctctccctttctctatctgctggatgcatgaacaggattatgaggatctagagactgtggagcataagacagcatgagcatgttcaggtgaggtgtctcatgcctgtaattctagcattttgggaggctgaagtggagggatcatttgagtccaagaatttcaaccagcctgggcaacttagtgagacctcatctctatgaaaataaaaatatacaaaattagccagatatagtggtgcatgtctgtagtcccagctactcaagaggctgaggcaggagaatcacttattcttaattctctctccctttctccatctgctggatcatggacaggattctgaggatctagagaatgtggagcccaagacgggagaagcctgcatttctgaatgacagtgtggcactgtgccctctttctgcagaccagcattggcctgtgacatgagcaagaagtaaacttttgttgtggctaactacttagaccgtggacatttttgttgcagtggttggcctactctgattgataaatgtgtgccagctgctatggcttgagctttatcatagtggggaacacagtatggtgaagtcaatagatcttagcagagtatcagctggattgtcagataaatcttctcctagcactatccctgtctctttcacaacagagactggcaaattctcaggttcactaattaaactatcatgctttttataccctttctttaccttctaatagattgagtggcacaggtaaaggagtggtgagatcactgtgtatagaaacaacaggaaatttggatctggctaatcctgctatataagggggagtcagttgcttcccatttgagagcttggcatctgcctttgctcatttttttctcaaaatcaaaggagctgtccacagcctcaacagtgattcttctccttttttttttttgagttggagtctcgctctgtcgcccaggctggagtgcagtggcacaatcttggctcactgcaacctccgcctcccaggttcaagcaattctcctgccttagcctcctgagtagctgggattacaggcgcttaccaccacacccggcttaatttttgtatttttagtagaaatggggtttcaccatgttggtcaagctggcctcgatctcctaacctcgtgatccacccgcctcagcctcccaaagtgctgggattacaggcgtgagccactgcgcccggcaacagtgattcttctttatgaacactctcactaacagcattatttccttctcctaggaggaaattatgtccttgaagtgaattggggatcctctctcctcaacagaaatcatgggcttgcattgttcaggtggtcataaatggagttattcttcccaacttttcttttaaaggtccagtaccagtattcaccccaagagtgtattacgccatggctgcactgagttcactgttacacaaatgtggcacaatctcacctcattttctttctttgcgcatgctggtttctttttgtcttttcttttcttttttttttttgacaagtgtcttgatctgttgctcaggctggagtgcagtgaagtgaacatggctcactgcagcctcaacctctcctgcctcagtctctcaagtagctgggactacaggtgtgcatcatcatgtctggttaatttttatttatttattaattattattattatttttggacagagtcttgctctgttgcccaggctggagtacagtggtgtgatctcggctcactgcaagctctgcttcccgggttcatgccattctcccgcctcagcctccccagtagctgggactacaggcacccaccaccaagcctggctaattttgtttttgtatttttagtagagatgggctttcaccatgttagccgggatggtctcgatctcctgaccttgtgatccacccgccttggcctcccaaagtgctgggattacaggcataagccaccgcgcccggcctattatcatgattttttgtagagatgaggtttcactaagttgcccaggctggtcttgaactcttgggctcaagtgatccctccacctcagcctcccaaagtgctaagattacaggcataagacacctcatgtggacaagtacatgttgttttccttgcttggattgttcttttctgatctttttccccttgaaaatgtctactggctgttaaatgtctttggaaactctcaagtaatattgtggctacagttcccctagcactttgtttatttattttttattttttttatttttttgagatggagtttcgctcttgttgcccaggctggagtgtgatggtgtgatctcagcttactgcaacctctgcctcccgggttcaagtgattctcctgcctcagccttccgagtagctgggattacaggcatgcgccaccatgcctggcctatttttctttgtatttttagtagagactgagtttctccatgttggtcaggctggtcttgaactcccgacctcaggtcatctgcctgccttggcctcccaaagtgctgggattacaggtgtgagccaccacgcctggcctgtttatattttttaataagtattttgggttatgcctccaggaaggtgactacatttaatctttttgcagcaatctgaatcccagtactttcagacatatagtgtatgctctataaaaatttgtggaatgaataattgaaagtgagtagggaaagacttgagtggattttgtcttagagcagtatcatccacgtggtccccaacatatatgatggaataacttcttttaggactcgatggtggccataggtatctctttgttttgggcatgaacaagctcctttcccattttgagaaagtgaaatttaatgtctatctttaaatatgggtactatcttacccttattgaattaaaatcctttctgattgtcctagccgtctcttcagtttcctcatggccaacttcatttcctgattcctcagcgtgtaaattataggattgagcaaaggggagatgacagtgaaggtgacagagatggcagtgtctgtggggagggcagtgaagggccgggcatagacatagatgcagggcacgaaatgcagggtcaccacggtgatgtgggaggtgcaggtggagatggctttcctcctgccttccccagtgtgagacctcagcatcatcaagatgaccgtgtaagatatgaggagaaagaagaatacaaaccaactgactaacccattatttgaaatcatcaggagctccagagtgaaggtgtcagtgcaggcaagtttgaggacctgggggacatcgcagtagaaagtgtcaagaacattgggtccacagaaagggagtgggagcaatagagaaatctgcgctatggagtggacaaagccccccacccaggaagccacgatgaggcctgtgcatcgccccctactcatgatggtcatatagtgcaggggcttggagatggctatatagcggtcaaacgccatcacagagagagaaaaaacgtctgctccccccagaaggtggaagaagaacatttgagtgacacagccactgaaggagatggtttttgtctctgatagaagatctatcaggaccttaggagctgtgatggaggaaaagcagatgtcaagaatagacaggttgcggagcaggaagtacatgggcgtatgaaggtgagattcacaggtaactgtaaccatgatgaggaagtttcccattagagttgtcatgtacaccaaaaacaggaaggtaaataagacctggctcagttctcgggactgagtaattcccaggaaggtaaattctttcactctggtgtaatttctctgatccattgaatcacagatcctttatcaggttcatcttgtgtctgcaagtcagtatgccaccactggatgaaagattacccaggtttttgattcagtcatcccaggagacaaagttctctcactgctgctgctcttttctttgcttcttaagagtcttgacttccataggaacattctacacatttgcagcatttctcaaaattcagcacaaacagcttttcagtttcagaagttcataggcactaatactaactgctggtttaatctttaagtgggaaattgatcctcttatgatgcctcagctgcattttagaagaagtaggtactggggaaattct

SEQ ID NO: 14167 - RNA, 2961 nt, Homo sapiens
  source 1..2961: mol_type = other RNA
gctgggattacaggcatgagccaccgcagctggctaacccctctggtttcattagacctttgcccagtcttcttgtgcgatgtcacagaaacattggttcagggacaactttatgtttttgaacttttatttatctatttattttgagacggagtcttactcttgttgcccaggctggagtacagtggcgtgatctcggctcactgcaacctctgcctcccgggttcaagcgactctcctgccccagcctcctgagtagctgggattacaggcgcccgccaccatgcccagctaatttttttacttttagtagagatggggtttcgccatgttggccaggctggtcttgaactcctgccctcaggtgatctgcccgcttggcctcccaaagtgttgagattacaggcgtgagccactgcgcacggacgcttttgaacttttatttagactgtcagaatgtttggttggggccaaataaaagaagttgggaaggactggaacaaaacatgtttgtaggctggctctatggacttttgacagcatgctcctggcggaagaaaagttaagttttgcacccgctggagacagacactgacgtctcaagggggaaacagccacattcctgattatttcaagcagatggatggggaagggctgtgtgtcaatctgaaagagcctggatacatatctggggtgttctccaacaggcactgaagaagaatctcccccttctgtaagacactctccgtcagagactgatgttcatctatatctttcttaaattgccggtaaagctgcagagaagacttgagacttgtaagattggacctggctgcagtcccgtggtcagtaacatctgcaacattatacagccagcagatcagctcttccagctgacagcaaaatgtcttcacacattgcaccagtgattcttttccctgttctcctcctttcctgggaagctgcccttcaacatctgggtctgagaatggccaccggtccaacctagctggcaaggaggggcgtgttttcagcagtccagaggagaccccgagggcctggctgctccccagactgccttcccctgcggagtcgtgggcacggacgaaggagcgcaggaaacagggattctggccctcaggatccccagatccttggagggcagctccagggggaagctggctttggctggagcttgaagggaaggaagctggcccatcactgtctgacacttccaaggggctctgccctttgatatccccagtgggcagggtaaccaaggtagaaatggatcctagatacgaaaccaggctagaaacctgtgtcagccgagcggggagggcaagatactcgtcatcactttccacttcctcttctgatttccacctagactctgtgcaggtagggcgccgggcactctggctggtcctcttctccctctctggcctgggcgagggccaccctctgtcccgtgtccttagctggggagagcccatatcaaggtgcttgcctatagtcagccggtccttcgcacccctcagggctggctctctgcgctcccaacgagcatccctactgcctggggctctgggggtagatgcaagttggctccaagatgccaagcccatgccaccctgtttctggggtactctggagggccactgcttaaggcttggctctctgggcccagaaaatggcagggcagtggcctctgctggtgggcagttgggggagacattagtaggtgatttgagggtgcttgctggagagacagagaagctatccaggtctaccccggagtcctgcaggacagggtcagctggcacacggctatcaaggtgctttgggagctgaggcccgggcctcagtgggtaagtatagtcaagcagatcttcatactctttatttgggttccagagaggggagtggcggtcgggtgatggaggcagggaatctggcagcacacaggcccagtactcagcctggaaggagaggcgtctcctgcctagcccagaagcatcacccccagagaacacaggctgtggtgaccactggggccgaggtcctagccccaccacagaggaaggttcctgggggacgaccggctccagggaggaggagaccttggccagagaaccaccacgaggctccgccctctcctggtgaccctggagactgctgcctgtggaggaagcagagatgctgcagctggaaggctgagctgcggaacctgggctcagcacggacttccactgtgacaggcaagagagacctgagctgtgaggctgctggctgaggtccagtgcctggggcaaatctgctagggatggatcatcttcggtatcagcatcatgtcctgagcaaatagttgttgttctgggaaggctcagagtctgagggaactcctcggaggaagaaagcttggtcttctccacctggctttccccggagagcagaaggtctccagaccccatggtggcaggaggcaggccactgagtgcaggctcagacctctcagctacgggctctctgttggcatcactggcctgtggctggtgggctctagaggggccgccagggtcagtcccaatccagcaagtaggggcaggtatcccttctgccccccatacaggggagatgagccctccctcagcttccaggcgtgggggctgctccccactcatgggccctgggatgtccagctcccgctccctgcagctccctctcccataggactgggcctttgtgtcttcagatgcttccgcttctgccttttcttcacccagggccattgagactccctacctaggtcagggttctgctgaagacttcagcttccgcaccgcgaacgcttcgcacgtccggagcggtctcagcagccccatgcgctggccccgagctggcggaccctgactgcaactgcggccctccaaccgcagcccaaaacgcgcagggcaggac

SEQ ID NO: 14168 - RNA, 601 nt, Homo sapiens
  source 1..601: mol_type = other RNA
gctgggattacaggcatgagccaccgcagctggctgagcccatattttgttccaataaaggttcagtcatgcccttccattttttgtccagtgaagtgtgtcacccatgctgttctctgcaatatgtgccaccaggtgtaagagttgacaccatcctcatctttccaaatttgcagacatggtacaagggcttacgatagattgtgttgaaagttgacatcagtgaaggcacaagatgttacggggaaaaagagcaaagtgatctgacctactttatggagccaggaaaggcattagagggtagacgtggtgggtggcgtttaatctgaaacctcaaccccctcctcctggtgagagagccccactgggttccgcagagaagaggaagaggatgtgactcaaagattctgggcttccttggttccctgggctggaagtcagagagataatggaatccaggtgtgtgatctgcatgcatgcaggtttattttttttctctttttctttccaaagcagagaaggtgaggggtcatttctactctgggagagagcccccgaggtgtcagctgtggcggagtgctggcggcatctacagtggggg

SEQ ID NO: 14169 - RNA, 4712 nt, Homo sapiens
  source 1..4712: mol_type = other RNA
gctgggattacaggcatgagccaccgcatccagcccctgcaggtgtttcttaggaacgggctggtgccaatcacatccagattcaaacctttaagactaatgtaaccaaaaccatttacccggcaaacggctatctgcattgccaaactgaagaaacagcagcagatgtatacggcacacaagcgccctagttaaaactattaatctccaaatttgctgacaggaagaatgcagcaaggctagtgtgtgtgtgtgtgtgtgtgtgtgtgtgtgtgtgtgtgtgtgtgtgtgtgtgtgtgtgtatcaaatggccttaacattaaaggattatacttttaagaattttttaaatgttatttatagtttcaagataattaatggttcaattagcattaatctaatagagaaaagttcttagaataagagcttgcataaacaatctgaataaaatcttgactgcagtgtaaatttgcttcctttgaaaattttttaaacttacattatgtggtgtttttctttccctaaatgttatatataaataataacatttaatatttatggggaacttaagaaatatatatcaagcactgcttttttcattatctcactgccatctctaaacaacatagaatgcaggcacctctaaatagtactcccttgtacagacgggtcacagagggttcaaggtcacagagctggtaattgggagaacccaaatctgaacccttgattataaaatagctgcaatattcacattctaacttcattctcttatatcaattgagataaaatattcaatatcatccaaagttcctcaactagagaaatacagacaaaaaattctgactttataagaaatacaaatatggaagttaatctctctgaccgattagctcaagaaccaaattccagtaaagttactttgtccaacatctgattactgggcaacagactcttacttcaatttgtcatatttacctatatgcaaaataattcttacacgtatcacagacatgttgcatgcccctaatactgtctttaaagctcttcattttccatcttttatattctgcacttggcatgtgaaactgttaaaagaatttaaggcaattataggaatgtcaaggcaagggagaaagaaactggacaaatactataatggtacaaagttccttctcatcctttacccaccctcctcaaaacacaggggtcagtgctaattttaccttaattacattcatgctggtaacctaggagaagggcttaaaaaatataacaggaaaaatgagggtcatcaatcactgtcacaggtatttaaggagccacatggaacactctcaattattcatggacatggcagacgaagaaagcatggatgagatgaaattcttaaaaattcattgtaactaatggtttcaatgtcttgtcccaccaaacctcccatcagaaaaagctaacaagagtcctaactgtcaccactgggtttttccttcctcttttcctcctctgatggccaaccacagagtggacgataaatgggagaagagaaacagggtctgggcaatccacaaactgggtagcaggcccagacacaccagttaacagtcaagagttgactatatcacaaactatgaatggtgtattacaacaaagcactgttgttgcttttgatattgcaaaaaattttaatggttaaatgaaaaggcaattttagaatttaattttctatcactgaattttggaaccctcagctctgcataggaatttttgtagcatttaaataatgatcattcctatcaattctcaatctgatgatagctgagaggatcttcaatcttaaaaaacaaaaaagcaaataactgcctttcccccccaacaaatgctatttttccttatagctttctcagaatttatactaatcatgaaaatgaagcacttacaggtgtaggctgctcttattaaagggaactgtcgacctccagacaagcaagacccagaggatcgatgagtcagactgaagtttactatacatacatatgtctttctgagcatatctctacaaatgtctggctttagatgaagaaccaggagaaaaccatgaaagcactaagatctcaaaagaaccaaaatgaaagcttagagtgtgattgtttttcaaaagttatatcctatgtgttgatccaaaaatgaaaaggatatgggatataagatgaactttgagtaaaagtaacttgatggtgaataaggcttagtgggcatacctgatacctggcggtctgattttcagaactgggatgtcaatactgatgtaataatcttgagctcctggagctgatcaggctcgtagagtttgggggacagcgcctgagccaggaaggcatctagctcctgacgccgaaggatgcgtgctcccggccactgcaccatgtaccgtaagacgcagcagagcaccatgaggtgagtgggcacgttggcagggttgagcatggctggggtgtccgacctcatgcaggccaggaaggccctcatcctgcggttcttgtcctctaccgccttacccaaccacagcctcttcaggttggggcaggtccactccctgaaggcaagagcttcaaccagttccggggtttgaggagactttcctttgtaagctgcccattctttaatgatcactggtgaaaattctggtggaagtctgttctttctaaaagcaagtctctcagttttctttctgctttctgccaaactaaacaggactccgtaaacatactgacgaactggcctatagagcagagcggccggaggcaggtccttgttggcttcatcttcaatagaaacagcaattttgatttcacccttcgtcaggacatggaagatgtaggggtacatcagccccttcttgtgcctgtgctcggccactctcagcacctcaggtgcgacggggggcaggggaggtgtggtgatgtccatgtggttcctggtgggcatcgacaggaggcacgggattggctggacagtgcccatctggcttcccttgccttcggctagttggcttcctgaagaggcagtggacgagccttctgcctttgtttggtctcctgggtctcctcgtgcctgaggctctgagtggcttcccgtcttctcccagccaatcttgttcccgctgatatggccatgcctcaggatcctggagcagagcacgatggaattctctttgtgaaacacaaagtttttttgcaagtagagttggaaaggctttgtcgcccctccgctgccctcgtcgttgtcggaagatgacgatgtagaagagccagggaagtaggcggaatccacgtggttggggctgccgctctgggccgggttgatgggcgaggaccgctcatacagcggcgtgtgcttcccttcgtgaggaatgttgctgtagctgttctgctccgtcagattcttcccgctcgtgtccaaagtgagaggtgctggctcagagaggctgtacgggtatggaccctggcccggggcgccccctgggctgggcacctgtggggccacgggctttgcttgcagagaggtctgcggaatgttgagcatctgaggaggaacatgcggcggcaccatcccaggcattccaaacggaccgggtctggctgctaagtaatgtggtggatgaaatgacataggcttactagtcgctgaataatatccaattgctctcttaaatcgaataactttgtcatctgttctagactgtgaatgctggaaaacatctttagctatggcatccaagtcagaggtgtcctgaatgttgcgtacatagtcagcaacggctttgatcactacgtcgcaaggtggcaagaccagctggtgggcccggacctttagtgaggctagtggatgttctggaccaagtaaactccagtgaaaggaagccagatcttcatcaggcagaatgtgatttcctaagagagcagcaaaaataggaaaacgatttggattcaggtccagttgcttggcaacttcatgcatcagatattggcttgtggtgagacttttcccgttccggctcagttttagggcatgggcactgaaatagtaggggatgttgcacagtgcataatcagagtcatacgcaaccaagccatggaaaccattctctctgcagaaaccaatcacttcctgatggtgatcctcaatgctctgtgcaaccttgacgtggaagcggatgagcgccaggcggatgcagtgggccatgcagacgggcggcaggaaccagacctttggcggcggggtgcccttgttctggacatggctgacgatctgctgtgccgtctggcgctcgttgccctgccgcttgacccactcgtgcagccgggccttctcgagcgcgccgttgaagaagacgaagagctcgatgttgccgccgaagcaggccttggccagcgccgccaggtagccaagcatgtggttccactggccgccgctgacccagtcggtgtagaagccgccgtagaggcggtgcaggcagttgtcggcgtccaccagcaggcgcagcggggtctgcgggggccgctgccgcccgccgcccaccaggctgccccgggccagcttctgcagctccaccggcaccacggcgctcgggcagtgcttctcgatgtagtcctggaagccctgcacgcccatggcggcggcgggggcgcgggcgcgggtgcgggcggggg

SEQ ID NO: 14170 - RNA, 1700 nt, Homo sapiens
  source 1..1700: mol_type = other RNA
gctgggattacaggcatgagccaccgcatccggccagatttcaggtgcttttaaaaagtaactgaaattttatttttacttaattcctttatttatatatatatatatacctgaaattaaggcaaaaagcatgatatgagacccaaaaaagctcatatcctactcaactaaaagtgtttaggacctaaacagggcaaaagatttaaatagcactaacagctcaaggaatgtataggttaaaccttttgttttacatccagaaaattagaaaactcagctaaacattgtatatatcacaaggttttaaaaataatttgtaagatttaatcttaccaagaaagcttactcatttaaagacttctttataccggcccttcatatcatcagtggaaactgtttattaaaagggaggagtatgggatacacaaatagcataaatcgaaatctcacacttaatcctttaatgttaattgcatttcagactgagtaaagtctgactaaaaatcacagcaatgggacaaagcactgctttgttttaaaactgcacatgtgctttctcccctgagaacctttggcttagactttttgtacagtaagacatttcattaaatatggttagatttgcagtctaagaccttaagtgacacactcaatgacaacattcttataaattatagccaattataagtcctccttctggtttctcttctgtgcttcgtaaatatgtacatctttttcaggatcgtagtgaacctttctcacagtaaattgcctctccagcattgctaagaagttgttatcccgttcatagcgaattcggcatgctaaaagaatcacagagtgattgctacagagatgttccagtgtctgaagaagatctgtgaatgtttcttctaaatatatgatatcagcaccaagtatcaggtcaaattctccaggagaaaaactccccaaattttgtccccaagtcagctccttaacaacagttttagtttggatatgaggaggtaagttggcttgaacgtttgatttaagaaattctaatgctacttttcgatccgtgatagtcacatgagcacccagcagggcagccactatgcccaccagccccgtgccagcacccagctccacggcagagcggcccctgagctccacagctcccatctccaggtatgtggaaagaacgatggccgcatcccaaaccaccgctgcgactcccaggtgtctccagtcctgccggatctggatcgtgtggtttgcaaaggaaaaagttgcaagaggcttgtggaatttctgcaacccaaattccgtggtctcctcatagggcacgagggccattccgcctgcaccccgccctctgctcagacccctctcccgggacgaccagtgcgcccttcctgcccgggggccccggagctgcggcaaccctccaggggtgagagggagaccaggcgaggggggtcacagggcctcttaggatccccaggccatacggggcgccgtgagctgcccggcggagcacccagggctcgcccaggccgggctgaggcgccgccacgccggtacttacggcccgggaggcggtcccgcgtggagcgcgcgctccgctttccccgccccgggctggctgcgaaaaccgccggccttaaagagcccgcgacgcgggggcgggcggccccggcccggagccacgcatttcc

SEQ ID NO: 14171 - RNA, 1498 nt, Homo sapiens
  source 1..1498: mol_type = other RNA
gctgggattacaggcatgagccaccgcatccggccagatttcaggtgcttttaaaaagtaactgaaattttatttttacttaattcctttatttatatatatatatatacctgaaattaaggcaaaaagcatgatatgagacccaaaaaagctcatatcctactcaactaaaagtgtttaggacctaaacagggcaaaagatttaaatagcactaacagctcaaggaatgtataggttaaaccttttgttttacatccagaaaattagaaaactcagctaaacattgtatatatcacaaggttttaaaaataatttgtaagatttaatcttaccaagaaagcttactcatttaaagacttctttataccggcccttcatatcatcagtggaaactgtttattaaaagggaggagtatgggatacacaaatagcataaatcgaaatctcacacttaatcctttaatgttaattgcatttcagactgagtaaagtctgactaaaaatcacagcaatgggacaaagcactgctttgttttaaaactgcacatgtgctttctcccctgagaacctttggcttagactttttgtacagtaagacatttcattaaatatggttagatttgcagtctaagaccttaagtgacacactcaatgacaacattcttataaattatagccaattataagtcctccttctggtttctcttctgtgcttcgtaaatatgtacatctttttcaggatcgtagtgaacctttctcacagtaaattgcctctccagcattgctaagaagttgttatcccgttcatagcgaattcggcatgctaaaagaatcacagagtgattgctacagagatgttccagtgtctgaagaagatctgtgaatgtttcttctaaatatatgatatcagcaccaagtatcaggtcaaattctccaggagaaaaactccccaaattttgtccccaagtcagctccttaacaacagttttagtttggatatgaggaggtaagttggcttgaacgtttgatttaagaaattctaatgctacttttcgatccgtgatagtcacatgagcacccagcagggcagccactatgcccaccagccccgtgccagcacccagctccacggcagagcggcccctgagctccacagctcccatctccaggtatgtggaaagaacgatggccgcatcccaaaccaccgctgcgactcccaggtgtctccagtcctgccggatctggatcgtgtggtttgcaaaggaaaaagttgcaagaggcttgtggaatttctgcaacccaaattccgtggtctcctcatagggcacgagggccattccgcctgcaccccgccctctgctcagacctcccctcctccatcggctgcttcgatagtgataacaatgggacagaacctgcccttagactgggtgttagcggtttgataaaccagaaatacatggtcgccgcagttccgtctccccgaccctggaagtg

SEQ ID NO: 14172 - RNA, 1514 nt, Homo sapiens
  source 1..1514: mol_type = other RNA
gctgggattacaggcatgagccaccgcatccggccagatttcaggtgcttttaaaaagtaactgaaattttatttttacttaattcctttatttatatatatatatatacctgaaattaaggcaaaaagcatgatatgagacccaaaaaagctcatatcctactcaactaaaagtgtttaggacctaaacagggcaaaagatttaaatagcactaacagctcaaggaatgtataggttaaaccttttgttttacatccagaaaattagaaaactcagctaaacattgtatatatcacaaggttttaaaaataatttgtaagatttaatcttaccaagaaagcttactcatttaaagacttctttataccggcccttcatatcatcagtggaaactgtttattaaaagggaggagtatgggatacacaaatagcataaatcgaaatctcacacttaatcctttaatgttaattgcatttcagactgagtaaagtctgactaaaaatcacagcaatgggacaaagcactgctttgttttaaaactgcacatgtgctttctcccctgagaacctttggcttagactttttgtacagtaagacatttcattaaatatggttagatttgcagtctaagaccttaagtgacacactcaatgacaacattcttataaattatagccaattataagtcctccttctggtttctcttctgtgcttcgtaaatatgtacatctttttcaggatcgtagtgaacctttctcacagtaaattgcctctccagcattgctaagaagttgttatcccgttcatagcgaattcggcatgctaaaagaatcacagagtgattgctacagagatgttccagtgtctgaagaagatctgtgaatgtttcttctaaatatatgatatcagcaccaagtatcaggtcaaattctccaggagaaaaactccccaaattttgtccccaagtcagctccttaacaacagttttagtttggatatgaggaggtaagttggcttgaacgtttgatttaagaaattctaatgctacttttcgatccgtgatagtcacatgagcacccagcagggcagccactatgcccaccagccccgtgccagcacccagctccacggcagagcggcccctgagctccacagctcccatctccaggtatgtggaaagaacgatggccgcatcccaaaccaccgctgcgactcccaggtgtctccagtcctgccggatctggatcgtgtggtttgcaaaggaaaaagttgcaagaggcttgtggaatttctgcaacccaaattccgtggtctcctcatagggcacgagggccattccgcctgcaccccgccctctgctcagacctcccctcctccatcggctgcttcgatagtgataacaatgggacagaacctgcccttagactgggtgttagcggtttgataaaccagaaatacatggtcgccgcagttccgtctccccgaccctggaagtgagcgacactgggggcc

SEQ ID NO: 14173 - RNA, 1476 nt, Homo sapiens
  source 1..1476: mol_type = other RNA
gctgggattacaggcatgagccaccgcatccggccagatttcaggtgcttttaaaaagtaactgaaattttatttttacttaattcctttatttatatatatatatatacctgaaattaaggcaaaaagcatgatatgagacccaaaaaagctcatatcctactcaactaaaagtgtttaggacctaaacagggcaaaagatttaaatagcactaacagctcaaggaatgtataggttaaaccttttgttttacatccagaaaattagaaaactcagctaaacattgtatatatcacaaggttttaaaaataatttgtaagatttaatcttaccaagaaagcttactcatttaaagacttctttataccggcccttcatatcatcagtggaaactgtttattaaaagggaggagtatgggatacacaaatagcataaatcgaaatctcacacttaatcctttaatgttaattgcatttcagactgagtaaagtctgactaaaaatcacagcaatgggacaaagcactgctttgttttaaaactgcacatgtgctttctcccctgagaacctttggcttagactttttgtacagtaagacatttcattaaatatggttagatttgcagtctaagaccttaagtgacacactcaatgacaacattcttataaattatagccaattataagtcctccttctggtttctcttctgtgcttcgtaaatatgtacatctttttcaggatcgtagtgaacctttctcacagtaaattgcctctccagcattgctaagaagttgttatcccgttcatagcgaattcggcatgctaaaagaatcacagagtgattgctacagagatgttccagtgtctgaagaagatctgtgaatgtttcttctaaatatatgatatcagcaccaagtatcaggtcaaattctccaggagaaaaactccccaaattttgtccccaagtcagctccttaacaacagttttagtttggatatgaggaggtaagttggcttgaacgtttgatttaagaaattctaatgctacttttcgatccgtgatagtcacatgagcacccagcagggcagccactatgcccaccagccccgtgccagcacccagctccacggcagagcggcccctgagctccacagctcccatctccaggtatgtggaaagaacgatggccgcatcccaaaccaccgctgcgactcccaggtgtctccagtcctgccggatctggatcgtgtggtttgcaaaggaaaaagttgcaagaggcttgtggaatttctgcaacccaaattccgtggtctcctcatagggcacgagggccattccgcctgcaccccgccctctgctcagacctgcccttagactgggtgttagcggtttgataaaccagaaatacatggtcgccgcagttccgtctccccgaccctggaagtgagcgacactgggggcctccaagcggct

SEQ ID NO: 14174 - RNA, 1619 nt, Homo sapiens
  source 1..1619: mol_type = other RNA
gctgggattacaggcatgagccaccgcatccggccagatttcaggtgcttttaaaaagtaactgaaattttatttttacttaattcctttatttatatatatatatatacctgaaattaaggcaaaaagcatgatatgagacccaaaaaagctcatatcctactcaactaaaagtgtttaggacctaaacagggcaaaagatttaaatagcactaacagctcaaggaatgtataggttaaaccttttgttttacatccagaaaattagaaaactcagctaaacattgtatatatcacaaggttttaaaaataatttgtaagatttaatcttaccaagaaagcttactcatttaaagacttctttataccggcccttcatatcatcagtggaaactgtttattaaaagggaggagtatgggatacacaaatagcataaatcgaaatctcacacttaatcctttaatgttaattgcatttcagactgagtaaagtctgactaaaaatcacagcaatgggacaaagcactgctttgttttaaaactgcacatgtgctttctcccctgagaacctttggcttagactttttgtacagtaagacatttcattaaatatggttagatttgcagtctaagaccttaagtgacacactcaatgacaacattcttataaattatagccaattataagtcctccttctggtttctcttctgtgcttcgtaaatatgtacatctttttcaggatcgtagtgaacctttctcacagtaaattgcctctccagcattgctaagaagttgttatcccgttcatagcgaattcggcatgctaaaagaatcacagagtgattgctacagagatgttccagtgtctgaagaagatctgtgaatgtttcttctaaatatatgatatcagcaccaagtatcaggtcaaattctccaggagaaaaactccccaaattttgtccccaagtcagctccttaacaacagttttagtttggatatgaggaggtaagttggcttgaacgtttgatttaagaaattctaatgctacttttcgatccgtgatagtcacatgagcacccagcagggcagccactatgcccaccagccccgtgccagcacccagctccacggcagagcggcccctgagctccacagctcccatctccaggtatgtggaaagaacgatggccgcatcccaaaccaccgctgcgactcccaggtgtctccagtcctgccggatctggatcgtgtggtttgcaaaggaaaaagttgcaagaggcttgtggaatttctgcaacccaaattccgtggtctcctcatagggcacgagggccattccgcctgcaccccgccctctgctcagacctggcgctgaatgtgcctctcgaccttttctatcatgtgctccgccgctctctgcctctgactttgtcgcttgcgcgttgtgcctgttttttaaaggtggcgcgttagcggatgatggagacagctcgctccgaagaaggcatggtcactctagtccccgcgtctccacggtggggtcagaagcggcgtaatagcccgcttggcggcaatcgagtggaaaagtcacaaaacccttttcaactaaagcacagt

SEQ ID NO: 14175 - RNA, 1744 nt, Homo sapiens
  source 1..1744: mol_type = other RNA
gctgggattacaggcatgagccaccgcatccggccagatttcaggtgcttttaaaaagtaactgaaattttatttttacttaattcctttatttatatatatatatatacctgaaattaaggcaaaaagcatgatatgagacccaaaaaagctcatatcctactcaactaaaagtgtttaggacctaaacagggcaaaagatttaaatagcactaacagctcaaggaatgtataggttaaaccttttgttttacatccagaaaattagaaaactcagctaaacattgtatatatcacaaggttttaaaaataatttgtaagatttaatcttaccaagaaagcttactcatttaaagacttctttataccggcccttcatatcatcagtggaaactgtttattaaaagggaggagtatgggatacacaaatagcataaatcgaaatctcacacttaatcctttaatgttaattgcatttcagactgagtaaagtctgactaaaaatcacagcaatgggacaaagcactgctttgttttaaaactgcacatgtgctttctcccctgagaacctttggcttagactttttgtacagtaagacatttcattaaatatggttagatttgcagtctaagaccttaagtgacacactcaatgacaacattcttataaattatagccaattataagtcctccttctggtttctcttctgtgcttcgtaaatatgtacatctttttcaggatcgtagtgaacctttctcacagtaaattgcctctccagcattgctaagaagttgttatcccgttcatagcgaattcggcatgctaaaagaatcacagagtgattgctacagagatgttccagtgtctgaagaagatctgtgaatgtttcttctaaatatatgatatcagcaccaagtatcaggtcaaattctccaggagaaaaactccccaaattttgtccccaagtcagctccttaacaacagttttagtttggatatgaggaggtaagttggcttgaacgtttgatttaagaaattctaatgctacttttcgatccgtgatagtcacatgagcacccagcagggcagccactatgcccaccagccccgtgccagcacccagctccacggcagagcggcccctgagctccacagctcccatctccaggtatgtggaaagaacgatggccgcatcccaaaccaccgctgcgactcccaggtgtctccagtcctgccggatctggatcgtgtggtttgcaaaggaaaaagttgcaagaggcttgtggaatttctgcaacccaaattccgtggtctcctcatagggcacgagggccattccgcctgcaccccgccctctgctcagacctggcgctgaatgtgcctctcgaccttttctatcatgtgctccgccgctctctgcctctgactttgtcgcttgcgcgttgtgcctgttttttaaaggtggcgcgttagcggatgatggagacagctcgctccgaagaaggcatggtcactctagtccccgcgtctccacggtggggtcagaagcggcgtaatagcccgcttggcggcaatcgagtggaaaagtcacaaaacccttttcaactaaagcacagtgggggaagtgaacacgtggcgcccgagtccaagtttttaaagtggggcgggggtcggcgggctctggctgcagtcggaagcgcggagctctgggcgtgcgctcggctccagccccggccccaggc

SEQ ID NO: 14176 - RNA, 1497 nt, Homo sapiens
  source 1..1497: mol_type = other RNA
gctgggattacaggcatgagccaccgcatccggccagatttcaggtgcttttaaaaagtaactgaaattttatttttacttaattcctttatttatatatatatatatacctgaaattaaggcaaaaagcatgatatgagacccaaaaaagctcatatcctactcaactaaaagtgtttaggacctaaacagggcaaaagatttaaatagcactaacagctcaaggaatgtataggttaaaccttttgttttacatccagaaaattagaaaactcagctaaacattgtatatatcacaaggttttaaaaataatttgtaagatttaatcttaccaagaaagcttactcatttaaagacttctttataccggcccttcatatcatcagtggaaactgtttattaaaagggaggagtatgggatacacaaatagcataaatcgaaatctcacacttaatcctttaatgttaattgcatttcagactgagtaaagtctgactaaaaatcacagcaatgggacaaagcactgctttgttttaaaactgcacatgtgctttctcccctgagaacctttggcttagactttttgtacagtaagacatttcattaaatatggttagatttgcagtctaagaccttaagtgacacactcaatgacaacattcttataaattatagccaattataagtcctccttctggtttctcttctgtgcttcgtaaatatgtacatctttttcaggatcgtagtgaacctttctcacagtaaattgcctctccagcattgctaagaagttgttatcccgttcatagcgaattcggcatgctaaaagaatcacagagtgattgctacagagatgttccagtgtctgaagaagatctgtgaatgtttcttctaaatatatgatatcagcaccaagtatcaggtcaaattctccaggagaaaaactccccaaattttgtccccaagtcagctccttaacaacagttttagtttggatatgaggaggtaagttggcttgaacgtttgatttaagaaattctaatgctacttttcgatccgtgatagtcacatgagcacccagcagggcagccactatgcccaccagccccgtgccagcacccagctccacggcagagcggcccctgagctccacagctcccatctccaggtatgtggaaagaacgatggccgcatcccaaaccaccgctgcgactcccaggtgtctccagtcctgccggatctggatcgtgtggtttgcaaaggaaaaagttgcaagaggcttgtggaatttctgcaacccaaattccgtggtctcctcatagggcacgagggccattccgcctgcaccccgccctctgctcagacggcccgggaggcggtcccgcgtggagcgcgcgctccgctttccccgccccgggctggctgcgaaaaccgccggccttaaagagcccgcgacgcgggggcgggcggccccggcccggagccacgcatttcc

SEQ ID NO: 14177 - RNA, 1527 nt, Homo sapiens
  source 1..1527: mol_type = other RNA
gctgggattacaggcatgagccaccgcatccggccagatttcaggtgcttttaaaaagtaactgaaattttatttttacttaattcctttatttatatatatatatatacctgaaattaaggcaaaaagcatgatatgagacccaaaaaagctcatatcctactcaactaaaagtgtttaggacctaaacagggcaaaagatttaaatagcactaacagctcaaggaatgtataggttaaaccttttgttttacatccagaaaattagaaaactcagctaaacattgtatatatcacaaggttttaaaaataatttgtaagatttaatcttaccaagaaagcttactcatttaaagacttctttataccggcccttcatatcatcagtggaaactgtttattaaaagggaggagtatgggatacacaaatagcataaatcgaaatctcacacttaatcctttaatgttaattgcatttcagactgagtaaagtctgactaaaaatcacagcaatgggacaaagcactgctttgttttaaaactgcacatgtgctttctcccctgagaacctttggcttagactttttgtacagtaagacatttcattaaatatggttagatttgcagtctaagaccttaagtgacacactcaatgacaacattcttataaattatagccaattataagtcctccttctggtttctcttctgtgcttcgtaaatatgtacatctttttcaggatcgtagtgaacctttctcacagtaaattgcctctccagcattgctaagaagttgttatcccgttcatagcgaattcggcatgctaaaagaatcacagagtgattgctacagagatgttccagtgtctgaagaagatctgtgaatgtttcttctaaatatatgatatcagcaccaagtatcaggtcaaattctccaggagaaaaactccccaaattttgtccccaagtcagctccttaacaacagttttagtttggatatgaggaggtaagttggcttgaacgtttgatttaagaaattctaatgctacttttcgatccgtgatagtcacatgagcacccagcagggcagccactatgcccaccagccccgtgccagcacccagctccacggcagagcggcccctgagctccacagctcccatctccaggtatgtggaaagaacgatggccgcatcccaaaccaccgctgcgactcccaggtgtctccagtcctgccggatctggatcgtgtggtttgcaaaggaaaaagttgcaagaggcttgtggaatttctgcaacccaaattccgtggtctcctcatagggcacgagggccattccgcctgcaccccgccctctgctcagacggcccgggaggcggtcccgcgtggagcgcgcgctccgctttccccgccccgggctggctgcgaaaaccgccggccttaaagagcccgcgacgcgggggcgggcggccccggcccggagccacgcatttccggtctcccggcacccagcctccggcaggtg

SEQ ID NO: 14178 - RNA, 1618 nt, Homo sapiens
  source 1..1618: mol_type = other RNA
gctgggattacaggcatgagccaccgcatccggccagatttcaggtgcttttaaaaagtaactgaaattttatttttacttaattcctttatttatatatatatatatacctgaaattaaggcaaaaagcatgatatgagacccaaaaaagctcatatcctactcaactaaaagtgtttaggacctaaacagggcaaaagatttaaatagcactaacagctcaaggaatgtataggttaaaccttttgttttacatccagaaaattagaaaactcagctaaacattgtatatatcacaaggttttaaaaataatttgtaagatttaatcttaccaagaaagcttactcatttaaagacttctttataccggcccttcatatcatcagtggaaactgtttattaaaagggaggagtatgggatacacaaatagcataaatcgaaatctcacacttaatcctttaatgttaattgcatttcagactgagtaaagtctgactaaaaatcacagcaatgggacaaagcactgctttgttttaaaactgcacatgtgctttctcccctgagaacctttggcttagactttttgtacagtaagacatttcattaaatatggttagatttgcagtctaagaccttaagtgacacactcaatgacaacattcttataaattatagccaattataagtcctccttctggtttctcttctgtgcttcgtaaatatgtacatctttttcaggatcgtagtgaacctttctcacagtaaattgcctctccagcattgctaagaagttgttatcccgttcatagcgaattcggcatgctaaaagaatcacagagtgattgctacagagatgttccagtgtctgaagaagatctgtgaatgtttcttctaaatatatgatatcagcaccaagtatcaggtcaaattctccaggagaaaaactccccaaattttgtccccaagtcagctccttaacaacagttttagtttggatatgaggaggtaagttggcttgaacgtttgatttaagaaattctaatgctacttttcgatccgtgatagtcacatgagcacctgaaaagaataaaaggcagtgtaccagcaagggcttcatcgatgacttaagtgccagcagggcagccactatgcccaccagccccgtgccagcacccagctccacggcagagcggcccctgagctccacagctcccatctccaggtatgtggaaagaacgatggccgcatcccaaaccaccgctgcgactcccaggtgtctccagtcctgccggatctggatcgtgtggtttgcaaaggaaaaagttgcaagaggcttgtggaatttctgcaacccaaattccgtggtctcctcatagggcacgagggccattccgcctgcaccccgccctctgctcagacccctctcccgggacgaccagtgcgcccttcctgcccgggggccccggagctgcggcaaccctccaggggtgagagggagaccaggcgaggggggtcacagggcctcttaggatccccaggccatacggggcgccgtgagctgcccggcggagcacccagggctcgcccaggccgggctgaggcgccgccacgccggt

SEQ ID NO: 14179 - RNA, 1563 nt, Homo sapiens
  source 1..1563: mol_type = other RNA
gctgggattacaggcatgagccaccgcatccggccagatttcaggtgcttttaaaaagtaactgaaattttatttttacttaattcctttatttatatatatatatatacctgaaattaaggcaaaaagcatgatatgagacccaaaaaagctcatatcctactcaactaaaagtgtttaggacctaaacagggcaaaagatttaaatagcactaacagctcaaggaatgtataggttaaaccttttgttttacatccagaaaattagaaaactcagctaaacattgtatatatcacaaggttttaaaaataatttgtaagatttaatcttaccaagaaagcttactcatttaaagacttctttataccggcccttcatatcatcagtggaaactgtttattaaaagggaggagtatgggatacacaaatagcataaatcgaaatctcacacttaatcctttaatgttaattgcatttcagactgagtaaagtctgactaaaaatcacagcaatgggacaaagcactgctttgttttaaaactgcacatgtgctttctcccctgagaacctttggcttagactttttgtacagtaagacatttcattaaatatggttagatttgcagtctaagaccttaagtgacacactcaatgacaacattcttataaattatagccaattataagtcctccttctggtttctcttctgtgcttcgtaaatatgtacatctttttcaggatcgtagtgaacctttctcacagtaaattgcctctccagcattgctaagaagttgttatcccgttcatagcgaattcggcatgctaaaagaatcacagagtgattgctacagagatgttccagtgtctgaagaagatctgtgaatgtttcttctaaatatatgatatcagcaccaagtatcaggtcaaattctccaggagaaaaactccccaaattttgtccccaagtcagctccttaacaacagttttagtttggatatgaggaggtaagttggcttgaacgtttgatttaagaaattctaatgctacttttcgatccgtgatagtcacatgagcacctgaaaagaataaaaggcagtgtaccagcaagggcttcatcgatgacttaagtgccagcagggcagccactatgcccaccagccccgtgccagcacccagctccacggcagagcggcccctgagctccacagctcccatctccaggtatgtggaaagaacgatggccgcatcccaaaccaccgctgcgactcccaggtgtctccagtcctgccggatctggatcgtgtggtttgcaaaggaaaaagttgcaagaggcttgtggaatttctgcaacccaaattccgtggtctcctcatagggcacgagggccattccgcctgcaccccgccctctgctcagacctcccctcctccatcggctgcttcgatagtgataacaatgggacagaacctgcccttagactgggtgttagcggtttgataaaccagaaatacatggtcgccgcagttccgtctccccgaccctggaagtgagcgacactgg

SEQ ID NO: 14180 - RNA, 1568 nt, Homo sapiens
  source 1..1568: mol_type = other RNA
gctgggattacaggcatgagccaccgcatccggccagatttcaggtgcttttaaaaagtaactgaaattttatttttacttaattcctttatttatatatatatatatacctgaaattaaggcaaaaagcatgatatgagacccaaaaaagctcatatcctactcaactaaaagtgtttaggacctaaacagggcaaaagatttaaatagcactaacagctcaaggaatgtataggttaaaccttttgttttacatccagaaaattagaaaactcagctaaacattgtatatatcacaaggttttaaaaataatttgtaagatttaatcttaccaagaaagcttactcatttaaagacttctttataccggcccttcatatcatcagtggaaactgtttattaaaagggaggagtatgggatacacaaatagcataaatcgaaatctcacacttaatcctttaatgttaattgcatttcagactgagtaaagtctgactaaaaatcacagcaatgggacaaagcactgctttgttttaaaactgcacatgtgctttctcccctgagaacctttggcttagactttttgtacagtaagacatttcattaaatatggttagatttgcagtctaagaccttaagtgacacactcaatgacaacattcttataaattatagccaattataagtcctccttctggtttctcttctgtgcttcgtaaatatgtacatctttttcaggatcgtagtgaacctttctcacagtaaattgcctctccagcattgctaagaagttgttatcccgttcatagcgaattcggcatgctaaaagaatcacagagtgattgctacagagatgttccagtgtctgaagaagatctgtgaatgtttcttctaaatatatgatatcagcaccaagtatcaggtcaaattctccaggagaaaaactccccaaattttgtccccaagtcagctccttaacaacagttttagtttggatatgaggaggtaagttggcttgaacgtttgatttaagaaattctaatgctacttttcgatccgtgatagtcacatgagcacctgaaaagaataaaaggcagtgtaccagcaagggcttcatcgatgacttaagtgccagcagggcagccactatgcccaccagccccgtgccagcacccagctccacggcagagcggcccctgagctccacagctcccatctccaggtatgtggaaagaacgatggccgcatcccaaaccaccgctgcgactcccaggtgtctccagtcctgccggatctggatcgtgtggtttgcaaaggaaaaagttgcaagaggcttgtggaatttctgcaacccaaattccgtggtctcctcatagggcacgagggccattccgcctgcaccccgccctctgctcagacctcccctcctccatcggctgcttcgatagtgataacaatgggacagaacctgcccttagactgggtgttagcggtttgataaaccagaaatacatggtcgccgcagttccgtctccccgaccctggaagtgagcgacactgggggcc

SEQ ID NO: 14181 - RNA, 1538 nt, Homo sapiens
  source 1..1538: mol_type = other RNA
gctgggattacaggcatgagccaccgcatccggccagatttcaggtgcttttaaaaagtaactgaaattttatttttacttaattcctttatttatatatatatatatacctgaaattaaggcaaaaagcatgatatgagacccaaaaaagctcatatcctactcaactaaaagtgtttaggacctaaacagggcaaaagatttaaatagcactaacagctcaaggaatgtataggttaaaccttttgttttacatccagaaaattagaaaactcagctaaacattgtatatatcacaaggttttaaaaataatttgtaagatttaatcttaccaagaaagcttactcatttaaagacttctttataccggcccttcatatcatcagtggaaactgtttattaaaagggaggagtatgggatacacaaatagcataaatcgaaatctcacacttaatcctttaatgttaattgcatttcagactgagtaaagtctgactaaaaatcacagcaatgggacaaagcactgctttgttttaaaactgcacatgtgctttctcccctgagaacctttggcttagactttttgtacagtaagacatttcattaaatatggttagatttgcagtctaagaccttaagtgacacactcaatgacaacattcttataaattatagccaattataagtcctccttctggtttctcttctgtgcttcgtaaatatgtacatctttttcaggatcgtagtgaacctttctcacagtaaattgcctctccagcattgctaagaagttgttatcccgttcatagcgaattcggcatgctaaaagaatcacagagtgattgctacagagatgttccagtgtctgaagaagatctgtgaatgtttcttctaaatatatgatatcagcaccaagtatcaggtcaaattctccaggagaaaaactccccaaattttgtccccaagtcagctccttaacaacagttttagtttggatatgaggaggtaagttggcttgaacgtttgatttaagaaattctaatgctacttttcgatccgtgatagtcacatgagcacctgaaaagaataaaaggcagtgtaccagcaagggcttcatcgatgacttaagtgccagcagggcagccactatgcccaccagccccgtgccagcacccagctccacggcagagcggcccctgagctccacagctcccatctccaggtatgtggaaagaacgatggccgcatcccaaaccaccgctgcgactcccaggtgtctccagtcctgccggatctggatcgtgtggtttgcaaaggaaaaagttgcaagaggcttgtggaatttctgcaacccaaattccgtggtctcctcatagggcacgagggccattccgcctgcaccccgccctctgctcagacctgcccttagactgggtgttagcggtttgataaaccagaaatacatggtcgccgcagttccgtctccccgaccctggaagtgagcgacactgggggcctccaagcggctcgcgggga

SEQ ID NO: 14182 - RNA, 1673 nt, Homo sapiens
  source 1..1673: mol_type = other RNA
gctgggattacaggcatgagccaccgcatccggccagatttcaggtgcttttaaaaagtaactgaaattttatttttacttaattcctttatttatatatatatatatacctgaaattaaggcaaaaagcatgatatgagacccaaaaaagctcatatcctactcaactaaaagtgtttaggacctaaacagggcaaaagatttaaatagcactaacagctcaaggaatgtataggttaaaccttttgttttacatccagaaaattagaaaactcagctaaacattgtatatatcacaaggttttaaaaataatttgtaagatttaatcttaccaagaaagcttactcatttaaagacttctttataccggcccttcatatcatcagtggaaactgtttattaaaagggaggagtatgggatacacaaatagcataaatcgaaatctcacacttaatcctttaatgttaattgcatttcagactgagtaaagtctgactaaaaatcacagcaatgggacaaagcactgctttgttttaaaactgcacatgtgctttctcccctgagaacctttggcttagactttttgtacagtaagacatttcattaaatatggttagatttgcagtctaagaccttaagtgacacactcaatgacaacattcttataaattatagccaattataagtcctccttctggtttctcttctgtgcttcgtaaatatgtacatctttttcaggatcgtagtgaacctttctcacagtaaattgcctctccagcattgctaagaagttgttatcccgttcatagcgaattcggcatgctaaaagaatcacagagtgattgctacagagatgttccagtgtctgaagaagatctgtgaatgtttcttctaaatatatgatatcagcaccaagtatcaggtcaaattctccaggagaaaaactccccaaattttgtccccaagtcagctccttaacaacagttttagtttggatatgaggaggtaagttggcttgaacgtttgatttaagaaattctaatgctacttttcgatccgtgatagtcacatgagcacctgaaaagaataaaaggcagtgtaccagcaagggcttcatcgatgacttaagtgccagcagggcagccactatgcccaccagccccgtgccagcacccagctccacggcagagcggcccctgagctccacagctcccatctccaggtatgtggaaagaacgatggccgcatcccaaaccaccgctgcgactcccaggtgtctccagtcctgccggatctggatcgtgtggtttgcaaaggaaaaagttgcaagaggcttgtggaatttctgcaacccaaattccgtggtctcctcatagggcacgagggccattccgcctgcaccccgccctctgctcagacctggcgctgaatgtgcctctcgaccttttctatcatgtgctccgccgctctctgcctctgactttgtcgcttgcgcgttgtgcctgttttttaaaggtggcgcgttagcggatgatggagacagctcgctccgaagaaggcatggtcactctagtccccgcgtctccacggtggggtcagaagcggcgtaatagcccgcttggcggcaatcgagtggaaaagtcacaaaacccttttcaactaaagcacagt

SEQ ID NO: 14183 - RNA, 1550 nt, Homo sapiens
  source 1..1550: mol_type = other RNA
gctgggattacaggcatgagccaccgcatccggccagatttcaggtgcttttaaaaagtaactgaaattttatttttacttaattcctttatttatatatatatatatacctgaaattaaggcaaaaagcatgatatgagacccaaaaaagctcatatcctactcaactaaaagtgtttaggacctaaacagggcaaaagatttaaatagcactaacagctcaaggaatgtataggttaaaccttttgttttacatccagaaaattagaaaactcagctaaacattgtatatatcacaaggttttaaaaataatttgtaagatttaatcttaccaagaaagcttactcatttaaagacttctttataccggcccttcatatcatcagtggaaactgtttattaaaagggaggagtatgggatacacaaatagcataaatcgaaatctcacacttaatcctttaatgttaattgcatttcagactgagtaaagtctgactaaaaatcacagcaatgggacaaagcactgctttgttttaaaactgcacatgtgctttctcccctgagaacctttggcttagactttttgtacagtaagacatttcattaaatatggttagatttgcagtctaagaccttaagtgacacactcaatgacaacattcttataaattatagccaattataagtcctccttctggtttctcttctgtgcttcgtaaatatgtacatctttttcaggatcgtagtgaacctttctcacagtaaattgcctctccagcattgctaagaagttgttatcccgttcatagcgaattcggcatgctaaaagaatcacagagtgattgctacagagatgttccagtgtctgaagaagatctgtgaatgtttcttctaaatatatgatatcagcaccaagtatcaggtcaaattctccaggagaaaaactccccaaattttgtccccaagtcagctccttaacaacagttttagtttggatatgaggaggtaagttggcttgaacgtttgatttaagaaattctaatgctacttttcgatccgtgatagtcacatgagcacctgaaaagaataaaaggcagtgtaccagcaagggcttcatcgatgacttaagtgccagcagggcagccactatgcccaccagccccgtgccagcacccagctccacggcagagcggcccctgagctccacagctcccatctccaggtatgtggaaagaacgatggccgcatcccaaaccaccgctgcgactcccaggtgtctccagtcctgccggatctggatcgtgtggtttgcaaaggaaaaagttgcaagaggcttgtggaatttctgcaacccaaattccgtggtctcctcatagggcacgagggccattccgcctgcaccccgccctctgctcagacggcccgggaggcggtcccgcgtggagcgcgcgctccgctttccccgccccgggctggctgcgaaaaccgccggccttaaagagcccgcgacgcgggggcgggcggccccggcccggagccacgcatttc

SEQ ID NO: 14184 - RNA, 1718 nt, Homo sapiens
  source 1..1718: mol_type = other RNA
gctgggattacaggcatgagccaccgcatccggccagatttcaggtgcttttaaaaagtaactgaaattttatttttacttaattcctttatttatatatatatatatacctgaaattaaggcaaaaagcatgatatgagacccaaaaaagctcatatcctactcaactaaaagtgtttaggacctaaacagggcaaaagatttaaatagcactaacagctcaaggaatgtataggttaaaccttttgttttacatccagaaaattagaaaactcagctaaacattgtatatatcacaaggttttaaaaataatttgtaagatttaatcttaccaagaaagcttactcatttaaagacttctttataccggcccttcatatcatcagtggaaactgtttattaaaagggaggagtatgggatacacaaatagcataaatcgaaatctcacacttaatcctttaatgttaattgcatttcagactgagtaaagtctgactaaaaatcacagcaatgggacaaagcactgctttgttttaaaactgcacatgtgctttctcccctgagaacctttggcttagactttttgtacagtaagacatttcattaaatatggttagatttgcagtctaagaccttaagtgacacactcaatgacaacattcttataaattatagccaattataagtcctccttctggtttctcttctgtgcttcgtaaatatgtacatctttttcaggatcgtagtgaacctttctcacagtaaattgcctctccagcattgctaagaagttgttatcccgttcatagcgaattcggcatgctaaaagaatcacagagtgattgctacagagatgttccagtgtctgaagaagatctgtgaatgtttcttctaaatatatgatatcagcaccaagtatcaggtcaaattctccaggagaaaaactccccaaattttgtccccaagtcagctccttaacaacagttttagtttggatatgaggaggtaagttggcttgaacgtttgatttaagaaattctaatgctacttttcgatccgtgatagtcacatgagcacctgaaaagaataaaaggcagtgtaccagcaagggcttcatcgatgacttaagtgctgtggttgaagacggacggaaacctctgtcaatttacacagactttcaaccaccacccctgcccatgctccctgtcgaattttggaaagcagcagccagcagggcagccactatgcccaccagccccgtgccagcacccagctccacggcagagcggcccctgagctccacagctcccatctccaggtatgtggaaagaacgatggccgcatcccaaaccaccgctgcgactcccaggtgtctccagtcctgccggatctggatcgtgtggtttgcaaaggaaaaagttgcaagaggcttgtggaatttctgcaacccaaattccgtggtctcctcatagggcacgagggccattccgcctgcaccccgccctctgctcagacccctctcccgggacgaccagtgcgcccttcctgcccgggggccccggagctgcggcaaccctccaggggtgagagggagaccaggcgaggggggtcacagggcctcttaggatccccaggccatacggggcgccgtgagctgcccggcggagcacccagggctcgcccaggccgggctgaggcgccgccacgccggtactt

SEQ ID NO: 14185 - RNA, 1639 nt, Homo sapiens
  source 1..1639: mol_type = other RNA
gctgggattacaggcatgagccaccgcatccggccagatttcaggtgcttttaaaaagtaactgaaattttatttttacttaattcctttatttatatatatatatatacctgaaattaaggcaaaaagcatgatatgagacccaaaaaagctcatatcctactcaactaaaagtgtttaggacctaaacagggcaaaagatttaaatagcactaacagctcaaggaatgtataggttaaaccttttgttttacatccagaaaattagaaaactcagctaaacattgtatatatcacaaggttttaaaaataatttgtaagatttaatcttaccaagaaagcttactcatttaaagacttctttataccggcccttcatatcatcagtggaaactgtttattaaaagggaggagtatgggatacacaaatagcataaatcgaaatctcacacttaatcctttaatgttaattgcatttcagactgagtaaagtctgactaaaaatcacagcaatgggacaaagcactgctttgttttaaaactgcacatgtgctttctcccctgagaacctttggcttagactttttgtacagtaagacatttcattaaatatggttagatttgcagtctaagaccttaagtgacacactcaatgacaacattcttataaattatagccaattataagtcctccttctggtttctcttctgtgcttcgtaaatatgtacatctttttcaggatcgtagtgaacctttctcacagtaaattgcctctccagcattgctaagaagttgttatcccgttcatagcgaattcggcatgctaaaagaatcacagagtgattgctacagagatgttccagtgtctgaagaagatctgtgaatgtttcttctaaatatatgatatcagcaccaagtatcaggtcaaattctccaggagaaaaactccccaaattttgtccccaagtcagctccttaacaacagttttagtttggatatgaggaggtaagttggcttgaacgtttgatttaagaaattctaatgctacttttcgatccgtgatagtcacatgagcacctgaaaagaataaaaggcagtgtaccagcaagggcttcatcgatgacttaagtgctgtggttgaagacggacggaaacctctgtcaatttacacagactttcaaccaccacccctgcccatgctccctgtcgaattttggaaagcagcagccagcagggcagccactatgcccaccagccccgtgccagcacccagctccacggcagagcggcccctgagctccacagctcccatctccaggtatgtggaaagaacgatggccgcatcccaaaccaccgctgcgactcccaggtgtctccagtcctgccggatctggatcgtgtggtttgcaaaggaaaaagttgcaagaggcttgtggaatttctgcaacccaaattccgtggtctcctcatagggcacgagggccattccgcctgcaccccgccctctgctcagacctgcccttagactgggtgttagcggtttgataaaccagaaatacatggtcgccgcagttccgtctccccgaccctggaagtgagcgacactgggggcctccaagcggctcgcggggacagcg

SEQ ID NO: 14186 - RNA, 1651 nt, Homo sapiens
  source 1..1651: mol_type = other RNA
gctgggattacaggcatgagccaccgcatccggccagatttcaggtgcttttaaaaagtaactgaaattttatttttacttaattcctttatttatatatatatatatacctgaaattaaggcaaaaagcatgatatgagacccaaaaaagctcatatcctactcaactaaaagtgtttaggacctaaacagggcaaaagatttaaatagcactaacagctcaaggaatgtataggttaaaccttttgttttacatccagaaaattagaaaactcagctaaacattgtatatatcacaaggttttaaaaataatttgtaagatttaatcttaccaagaaagcttactcatttaaagacttctttataccggcccttcatatcatcagtggaaactgtttattaaaagggaggagtatgggatacacaaatagcataaatcgaaatctcacacttaatcctttaatgttaattgcatttcagactgagtaaagtctgactaaaaatcacagcaatgggacaaagcactgctttgttttaaaactgcacatgtgctttctcccctgagaacctttggcttagactttttgtacagtaagacatttcattaaatatggttagatttgcagtctaagaccttaagtgacacactcaatgacaacattcttataaattatagccaattataagtcctccttctggtttctcttctgtgcttcgtaaatatgtacatctttttcaggatcgtagtgaacctttctcacagtaaattgcctctccagcattgctaagaagttgttatcccgttcatagcgaattcggcatgctaaaagaatcacagagtgattgctacagagatgttccagtgtctgaagaagatctgtgaatgtttcttctaaatatatgatatcagcaccaagtatcaggtcaaattctccaggagaaaaactccccaaattttgtccccaagtcagctccttaacaacagttttagtttggatatgaggaggtaagttggcttgaacgtttgatttaagaaattctaatgctacttttcgatccgtgatagtcacatgagcacctgaaaagaataaaaggcagtgtaccagcaagggcttcatcgatgacttaagtgctgtggttgaagacggacggaaacctctgtcaatttacacagactttcaaccaccacccctgcccatgctccctgtcgaattttggaaagcagcagccagcagggcagccactatgcccaccagccccgtgccagcacccagctccacggcagagcggcccctgagctccacagctcccatctccaggtatgtggaaagaacgatggccgcatcccaaaccaccgctgcgactcccaggtgtctccagtcctgccggatctggatcgtgtggtttgcaaaggaaaaagttgcaagaggcttgtggaatttctgcaacccaaattccgtggtctcctcatagggcacgagggccattccgcctgcaccccgccctctgctcagacggcccgggaggcggtcccgcgtggagcgcgcgctccgctttccccgccccgggctggctgcgaaaaccgccggccttaaagagcccgcgacgcgggggcgggcggccccggcccggagccacgcatttccggtc

SEQ ID NO: 14187 - RNA, 1553 nt, Homo sapiens
  source 1..1553: mol_type = other RNA
gctgggattacaggcatgagccaccgcatgtggcctaaaacgacccttaatacacaatcgtataactatgcagccaagaatctgatataaatttctcccgtttgcttatcacacgcagtatttcataaaaattactccaagtgcgttaacaaagttctaggaccattggtaagctgccccatattggatagtagagtttgttggggcatgggtcaagtactggactgtttcttccaggctgcttccctttgtaggagaaaaggtaaatgagggaagctctggtttcctgaagagattctttcacaggcaggacgtagcagagcctgcctcatcttcttcataaaagagcttttcggagcccaccagttggtcctgaattgtttcctttgcatgtccttcttccagtgttgccgaggcatccagcaaggtgctgatgtcagcggagtcagcgtcattcactggaaccagcagcctcctcctctgacacccttcagcttctgcctgttccagcagacgctgtggctcctctggcaactctacagtcacacctgttagctctgccagctcctgaccttggatttcctgctcagagacctgggtgggctgcaagtatctgttactcagggtctcgttgcgggcattgtcctccgccccaggaactcgtgaaggacatgaacgccgccggaaaaggactctgtgcacacgttcgggacctcctccaccacctgagcagatgcctttgaggtaagaaatgaatttcttccgacatgaaaagccaaccacaaccacagctaaaatgatgactaaaaccactatgatgataaggtagtgatagggagaggcaagcatccccaggatggtggtcactgtctcctccgctgctggggttttcccagtggaactggcagctgattcatttttgcacttgatgtcactccggggcgtacaattactgaccttgaccatccctctgggacaccctgttctacacgtccggcacatctcaggggagtttttatcctggaagcttcctttttcacactgacacacggtgtctctggtcgtggtacaggaacttttatttgtttgacctgatttacaaactgtacatagcaggcaagaaggcaaattgttggaagcaatggtgtaatccacaccctctgtgcacgggttacaggctccagtatattctgatctatgagatcctgctggacactcctcctccttgaggctgcgcctctgttgctgtggggccactgtctgctggggaacttcgtcctgccgggggatggtggcagagtcaacccggaccggcagcagaaccgcgacgatgaagacgacgaacttaaggatcttggggtccaggagccatggtctggttcccgacgctgtcctggctcctggatagcgccctgctcgagcgctcgaggcggtcgggacgctttgtccccaaagtcccatgagaagggaggagggtggatcgaaagcgccaaaaatcaatcagaaatcgtccccgtagtttgtgcgcgtgcaaaggttctcgcagctacact

SEQ ID NO: 14188 - RNA, 507 nt, Homo sapiens
  source 1..507: mol_type = other RNA
gctgggattacaggcatgagccaccgcattcggccaaccattctgagttcacttttttcatctcacaatggacaaatccaaccccagtctggaaggcaggagaccatggatacagttcccagggagtctccagagcagagagcaggatgcagaatggtgaagagtggattctgagacataaatggaaaatgcttataaggaatttgtttttgtaaactcttttcaatacgacctcacttctctggtcaaaagcaatccagagacttccctctcttctcttcctcttccctgactgccagtgggtggatggtttcctctctgtctgcgataagcactgcagaggactctcggagtttgtcctcactcctgatgccacacaccttttcttggcactttatctcgtcccaggggaagattcctgcagaaatttccttctctgtaatctcttgacagatggctctgctggcaagaacctcaatccttaggagtgcattaataggcttttat

SEQ ID NO: 14189 - RNA, 1483 nt, Homo sapiens
  source 1..1483: mol_type = other RNA
gctgggattacaggcatgagccaccgcccctggctggctatttatactctttccctaactctgtccctggggaaccttctcccctcacttcccctggagttccctcccgacaaaacacactcacttttatcttgctgatactgtggcctggggaactgctgagccagtgtcttgcacaggttcctttggctgaggatcgaggaaggccatgaattcctcatagcgacggagaaacagctggaagcgagccaggtatgagtcctcgttgtacggtagctgcttctcacgtaggaactgggacaccacgggcttcaccttcaggcacatgttatcagagagcctggggaatagatggtgttccacatggcagctgatgatcgagtggccgaacgcccagtccagcacgggcagccgggccaggttaagcacccccaggctcatcatgtgaatccgacggggcttgttgtcccgggagaacatgggcagtccgatgtgctggaagatgttgacgtggaggtaggggtgggccaacagggatctggtgaggaacatgcagcccagggctgagctggggttcttgaagcctgacacgttcaggagcagccagtagtgagaataaaggcccagagaaatcagggccagcgtccgcagggctgtcccgagctccaccttcctcagccgctcgacagccaccagtggagtggcgatggggaggaggaaaggagcaaggaacatgtagacatagcggttgaggcaaggcagcctccacgtgctggagtcccccaggcccaccacgttggtgtaggcatggtgcatcttgacgtgcccatgcgtggcgtgctctgcagtgaaggctgtgcacacctccacaaagaaaagcagccagatcttgctccagcgtttggactcggtgagggccccatgagtggccaggtggctgcccttgacagtgagtgtgtagtggcacacacccaagatggtgatgccggatgcaaagaccagggcattctcccagcgcaggcacaggaagcctgccggcaaggcgaagaggctgagcgcgaggatggcgcagtccacgccgtggcgctcccaccaggagctcgtcctcaccacgtcctgcaccagcacctccagctcccgcagcagcgcctcgcccccacggtgcgcgctccgcgccggttccatgggctccgtaggttccatgggctccgtaggttccatgggctccgtaggttccatgggctccgtaggttccatcggctccgtgggttccatggactctgtgggctcgggcccgacgcgcacggaggactggaggactggggcgtgtgtctgcggtgcaggcgaggcggggcgggccggggcggagtcacgcgccgcctggggacacccgcccccggggtcaaggtgcgagacaccctggctcctctgctgcgggcgctggcgacccaggcccggctcaggcgcgcgaccctggcaggcg

SEQ ID NO: 14190 - RNA, 1266 nt, Homo sapiens
  source 1..1266: mol_type = other RNA
gctgggattacaggcatgagccaccgcccctggctggctatttatactctttccctaactctgtccctggggaaccttctcccctcacttcccctggagttccctcccgacaaaacacactcacttttatcttgctgatactgtggcctggggaactgctgagccagtgtcttgcacaggttcctttggctgaggatcgaggaaggccatgaattcctcatagcgacggagaaacagctggaagcgagccaggtatgagtcctcgttgtacggtagctgcttctcacgtaggaactgggacaccacgggcttcaccttcaggcacatgttatcagagagcctggggaatagatggtgttccacatggcagctgatgatcgagtggccgaacgcccagtccagcacgggcagccgggccaggttaagcacccccaggctcatcatgtgaatccgacggggcttgttgtcccgggagaacatgggcagtccgatgtgctggaagatgttgacgtggaggtaggggtgggccaacagggatctggtgaggaacatgcagcccagggctgagctggggttcttgaagcctgacacgttcaggagcagccagtagtgagaataaaggcccagagaaatcagggccagcgtccgcagggctgtcccgagctccaccttcctcagccgctcgacagccaccagtggagtggcgatggggaggaggaaaggagcaaggaacatgtagacatagcggttgaggcaaggcagcctccacgtgctggagtcccccaggcccaccacgttggtgtaggcatggtgcatcttgacgtgcccatgcgtggcgtgctctgcagtgaaggctgtgcacacctccacaaagaaaagcagccagatcttgctccagcgtttggactcggtgagggccccatgagtggccaggtggctgcccttgacagtgagtgtgtagtggcacacacccaagatggtgatgccggatgcaaagaccagggcattctcccagcgcaggcacaggaagcctgccggcaaggcgaagaggctgagcgcgaggatggcgcagtccacgccgtggcgctcccaccaggagctcgtcctcaccacgtcctgcaccagcacctccagctcccgcagcagcgcctcgcccccacggtgcgcgctccgcgccggttccatgggctccgtaggttccatgggctccgtgggttccatggactctgtgggctcgggcccgacgcgcacggaggactggaggac

SEQ ID NO: 14191 - RNA, 1878 nt, Homo sapiens
  source 1..1878: mol_type = other RNA
gctgggattacaggcatgagccaccgcccctggctggctatttatactctttccctaactctgtccctggggaaccttctcccctcacttcccctggagttccctcccgacaaaacacactcacttttatcttgctgatactgtggcctggggaactgctgagccagtgtcttgcacaggttcctttggctgaggatcgaggaaggcctgccaaaagcaagctcaccctaaggtccccggggagagggcaccttggtgggcagagcctgaaggaagcaatagccaaggccgtgtggggctctcccaatgccagggaggtcccagccgagggagctgaccctgttctctctgtgccccctgctatctcccaggtggcccctgcacaggatccctcttcaccctgtcacctccctttaaccctaccaaggctcagatggagcagggggaaggacccagctctttagtcctgagatgaagttgctgaggtccagactgaccagaatgcacagccaccattaccgcttcacccagacacccctcaaaacccagaaaagcacgcaaggcaggtggcccccagaccccaggcctgagctcccctgcccccctgcctggccggtgcctccactctccaggtccaccaccagccactgagccacaccccctggaccagcagcagcaggagggccagggccaggccagggaggggcagggtggctgcaccggcccggcctcattacagccccacaagctcagtgatgggtggggcctgcaccatgaattcctcatagcgacggagaaacagctggaagcgagccaggtatgagtcctcgttgtacggtagctgcttctcacgtaggaactgggacaccacgggcttcaccttcaggcacatgttatcagagagcctggggaatagatggtgttccacatggcagctgatgatcgagtggccgaacgcccagtccagcacgggcagccgggccaggttaagcacccccaggctcatcatgtgaatccgacggggcttgttgtcccgggagaacatgggcagtccgatgtgctggaagatgttgacgtggaggtaggggtgggccaacagggatctggtgaggaacatgcagcccagggctgagctggggttcttgaagcctgacacgttcaggagcagccagtagtgagaataaaggcccagagaaatcagggccagcgtccgcagggctgtcccgagctccaccttcctcagccgctcgacagccaccagtggagtggcgatggggaggaggaaaggagcaaggaacatgtagacatagcggttgaggcaaggcagcctccacgtgctggagtcccccaggcccaccacgttggtgtaggcatggtgcatcttgacgtgcccatgcgtggcgtgctctgcagtgaaggctgtgcacacctccacaaagaaaagcagccagatcttgctccagcgtttggactcggtgagggccccatgagtggccaggtggctgcccttgacagtgagtgtgtagtggcacacacccaagatggtgatgccggatgcaaagaccagggcattctcccagcgcaggcacaggaagcctgccggcaaggcgaagaggctgagcgcgaggatggcgcagtccacgccgtggcgctcccaccaggagctcgtcctcaccacgtcctgcaccagcacctccagctcccgcagcagcgcctcgcccccacggtgcgcgctccgcgccggttccatgggctccgtaggttccatgggctccgtaggttccatgggctccgtaggttccatgggctccgtaggttccatcggctccgtgggttccatggactctgtgggctcgggcccgacgcgcacggaggact

SEQ ID NO: 14192 - RNA, 1756 nt, Homo sapiens
  source 1..1756: mol_type = other RNA
gctgggattacaggcatgagccaccgcgcacggcccacatctttcctctaaccttgcaggatatgacagctgagcagcatctttacttattaaaagtatttatttccagaaagagaaaattaaaactaagcactacttggcccaaaccaaacccctctagagatccagaacacacagggggcgctctttgggaggggtgctgagtgttagctgaaccccggggccctagcctttggctcccttcctcccttttgcaatcccccaagtgtgccgatgtgtgtgggatgtcagacaacacctggtctccctggctggggactgcttggacttgtaccgggagggacttcaggttttcagctaggttgatcatcctggaagctgaggaacttgaggtctcacaatgaagctgaggagaaggtcaggggtgggagcgcgttttctacttggtgccgctcaaggccatctgacagcctgagaggagtttggacacatttcacctcccctgcttccagcggccggggtgggttgcttctctagctcactggtccgagagttctctcctccactggggaaagatgcacggggacactgccagaattctagcctctcagataatggctaagggactaaagggacacactggagcctcattccgaggaaaagagccagacagaaaagatctgaacatctttgaatgcttgatgcctttgccaaaaaggcaattggaccccagtcaacaatgcaagtataaacacatgtgcacggaccatcaggggatcagggcaagctgggccaggctggcgaggttagctcagggagaaccaagccccagacgactacccgtggccaccccctgcattcattctccaaggcccacggtgggaggaaagggttttgctgttccctgctcttttggcagtgcacaggtcaggccctggcacagagtgggaactcagtatgaagtgaatgaacaggctgagttcccacccaaacttatgctcatggtgaagtgaaaaaggaaactggcaggcagggctggggcactgatcccagggctgaggtgcatctgatcggagtctgagaagcccagaatcctcagcattctgggaagcccctccttcaagggatgctctgcgtggaaagtgggctccctgtaggtatgttctagcaggattaagcaggattaacgaggctaagggccccgccacctggcagatgaaaatccttctccagtggagaggctgcatgtggccagactctctttgccctaactttgcagagcacccacctggctaggaaccttggagcgcatgttccttgtgtgcaagactcacagtaacccttgtttcagggggacacgaagagcaaagcttcgaagagctcttccatcctcccaggttatggaggaaggtgtggcggcttcttcctacgctacgatgctcccgccactttatgggacctggggagtgggaggggactgggtggaaggttaggatcgggatcgggggagcttttgttcctccatctcagttctaatggtcagccccagcaggaacaagccattctagccaaagccttgacaataatggaatttgtgttaataacctgggcacaggagagcagtgagggtagggacacaatgctttctttgtgcctgacagttgggtgccttgagccaaaaacctcctgaaactccctgaagataacgtgagcatttcttcccatgacaggggctccatgacttccaataacccag

SEQ ID NO: 14193 - RNA, 289 nt, Homo sapiens
  source 1..289: mol_type = other RNA
gctgggattacaggcatgagccaccgcgccaggccaatatttttaaataaaaaattacaaagctgtttttcttaaaatgttacaataaaattgtatctgtgtataaaatgtatcgcttccgccgcactgccgtctcggtcgcggttaccaccagtcgcagcgaggcgagccacggtgtagcggctccagcctccagcgtacggctggtgattacccattcctggtcctctaagccgggcactgagcagctccacaggaaaatacgggaacgtggaagagcctgacttcc

SEQ ID NO: 14194 - RNA, 6788 nt, Homo sapiens
  source 1..6788: mol_type = other RNA
gctgggattacaggcatgagccaccgcgccaggcccacatagtgcatatcctttaatacaacacactttggttttgatggggtgggggcagaatagtgaagcatacagcatgacatcattgaggatcacaggcctgaattccctcactgcattgccctgtgacctctgtctcccttgtgaagtgacaaggtcggtctaaatctttccttcagctttaggatttcaatgattctgtaagttttctccaataagaggttggttttgcaatagaattttaaagtcagtttgccaatgtattctatagataaaactgaattagtaagtggacctgttcaaagtctctctcaacaatatgtataatttaattagcagtttaaaaagtagaccattgattattagatcagccacctgtagaaaatatgcttttgtgcattttatggtgtgatattttctttcaaaagtgttactctgtgtacattatgtcattttggcataaatattttgtttatcagagcatctcattgcctaaacatatgagacaaaagataatatgattatcttatatattttgattagatctagtgaagttaaaactaatttttaaaaacctaaatcttgggttaatttgattcaaagcagttttaaccataaatttttaaaatcttactaagaatctctcatctctttattcatactcctggatgaagctaacagatgcatattcttcaagtgcagttctgattatgcatttttttgaatgaatacatttaatggttaccttactagtttttcaataaaataacaacctcttagcctggtagtcaagtccattttatttctatcttcatttctcctcagcattaattttcattatttttaatgcatcaaatacattttctaagccaccatttcttcatctagagatttggataataacttctacattttaggtaattttgaagattaagaaaaattaaatttctgtggcctagggtgagtacttaataaaccacaattattgattgttattattatttttgagaccccatgataaaaagaatatgcttactttaacagaagaaaacatggtttcaagtcctataccttacttgttattcctcatttcaggtaggttaattaatcttcctgtgctctcatttatttatttgtaaagtggttatagtagatgattaattaataagaggatggacttaaatacttgaggagaggactctagctaaaagcaccaacaagagtttgtttcccttttcgtttgttccatgtgtagcctatattttagctataggttaatcaccatttgtttaccatgtctttcctttcctaacactaaaagttttctcaggctagtccctcaatctacaatgtgctcctatatcctatctatcaatactttacctaaggcacagctgagatatttcccttatttaaagtcttaggatttttccaccaggaaatatcttccctatcctgtgtaccctcttttatctttccaaatatacttgtatatgtcctccttatttatatatacctcttgcttcccttacttagactataatacatgaaaggcagagatgggagcatcattcttcatatctcctaaatgacctttcccaatggcttgcagataagaaacattcaataaacttaggttaactacactatgatttttctgtatactttggtctctattttaaactccttgtctcccttctaaagtaatttctacatttagggacatttcacatcaagcagaatatataacatatttttactttccattgatctacccacatatcttttcaaatcttccctgaagttgtgctatcataggtagtcacagatgacagttggaaaagacaagagtaagtgcagctcaggggaatttcaatagtagactaacatgccctacttctggcatctgagaaaaaaacagcaagaaatgagaaagacagcactgttaacttggacctggaggttagagtgggctcatgagatgtggggttctctgtccactactctaaattgttaatgctatccttaaacaggtccaagaatctatgcttgaaaattagttcccttttctagtggtggttgtagtgatgacagtgatacttgttattttcatttatgtagcaatttcacttatatatatctcattttgacatggacaggaggcagggaaatactggttagaaaagggaggttccctagaaaaggccccaccctcaagcctggaaacttgcagccctaaatgagaataagcattcctgttttcgtgcccaaatgttgccttttccaagaccactctggcctgccatgcccctattctgtgcccatataaaccccaagctccataggcagagcagcagagcagtgtagcagagaaggaaagaagagaggaagtgtctgaacacatcaagagaagttcttctgggacgacaggcaaggacatcagccacgggacggctgaactcaggggaacatcatctgtccactccatctcctttccagctccccatcccatttagagccacctccttcactcaataaaatccccacattcaccattcttcaagtttgtgtgacctgattcttcctggacactggacaagaatttgggaggcagtgggtacgggaacccaaaaaggctgtcacactgactcttcactgagccgcttaacacttaagccattcttggatagctgggctaaaagagcactgtagcactcctggacactgccatgggtctggagcccaaaagtgctcactctggctcctgcacctgctcacttgtgtgctcccactcccataaggggtttgagcatgccacatccacgtcacaagtcccacaagggggtcagggaactctcccatttcaatttgaatagcaatccagttctcagaggtagttgttattacatctatcttacctatgagaacactgtggctcagagtgatgagccaaattggccagagtgactaagacactcatccgatagaagattctagacaaaatctcttctcctgcccccaccctccaccctccatctagttcactgccctcgataggttcttttatcccttcactttttaactggcatctctgaaatgctgaggggcaaaaaatgaaagaaaagataaaatactagtgccaaaggcaaagaagaaaataccaaacaattttagtgtaaaagtaactaaacgtccttatttctattaaaaaattagcttagatcggaactatataaggcagttttctcgctgtaagagaaaattttcagttgctgtaaagggtgacacaatgcgacccaagtgatctgtagacattttaaaaacagggctgagtccaaagtgccttttcagaaaggtgttagggcttcctcacaccacctggacaaaggggtatttgcttgtaagcaacctctacaagggtatttcatacaccctgtgtcctccacaatctgaagcttaaagaaatacaaagcagagtcagcggtgccctgggatgtttctgactttacaggtctgtcgagcttgggaagatactgacatttgttatatttttcttaaagccttttccagtaataaaaagtacatcttctcttcatttctaccagatgtatttttatttttgtccataaaaaatgtccaaagtcacacagtttacaatctgaatgcagtgatttctccgtaccaatacatatcacagaataaaataaaagttgctcactggcctgaaagatgggctaccataacatctgcctacaaagtgatttgctaaacagcattggaaatgcatatcccattaaaaatgtagcattagggaattcatccagaataatgacagaagcacaaaagcaggattaattagaaccctatttctttctacttaggcctcctatgtaacattatcttcatataattttgttttgtggtctaaaataattgtttctatataaaaatgattgtaatagctttgcagttgtatgtgttcactcttaaaaaccacagacttcatacacagaattactagaaaaactaaagtattaaccaagaaaaagattcaggctggtactggacacataaatattgttttatcaggaaaaaagaggagaatttggagagatgttacaccaacatcctccagcatttcatgttttccaatggaaactgaaacagtgtttctaataacttgattcaagggttattttacaaagaaaataaaatgcaaagatatattttacatcaataatttgaattatacaaaaaagaagaaactattgatcattttcttagaatgttactataatagctatttccctagaagaggtttcaatgcagtcaaattttgatcaggcaagtgggagaaggttaagaccttagaggcctatttcaggatatcagggaaaaggaaacttgtaaaataattgtaaatcagttttctaaactgataatgtagcccttatcgataatggtttctaacttactaatattcttgattcttttgagaaaagaagttatcgatgacattaaatggatgacattacttaaatgtcatcaaatggttaatggatgacattaaaatgtgtatcaaggtgattgtggccttcttttttaaataaaaatttttcctaaagtgtgtagattgttgaggattgtctgcttactgtgaaaagctgatgcctgtccacaagggtagcttggaggtgcccatcggaggaacatggggagcggagtgtaagcctttgggagcaccgtgctatgactgcagatgctccctggctgctcagagcctagctgtgactaagccaaggctactctactacctgctttcttcatgtcttcaatggcttaggactggcttcataactagcttctggttgttgctcactgacccacacaggccttgaacctgtgatcctgaccttgcttgttctaaggcctaataactatgagtggtgtctaatactcactgattcttgaaaggtcctgtagaacccaataagcttccctcaggcacttctgcacacactctgggacatcctttcagcaagtccattccagaggagtttgacatctgaccactcaaaaagccatggaaatttgctccaggcagacaacaggaccctctgttgggcttggccagtggtttctgcagcaatcgggttgtctggaccatttagctttttagcaaaacttcctgttcctacaaataatcccactaatcctctctctccccagctgcttccttgcctttcctgcttggctcccctctcataagcctctttctttctaattttttcagaggaacatattttacagtcccgttgcttcacctaccttgcccattgtccttgcctaaaattgtccttgactgaaatagtaagagatagttttcctctgctttttgaaatcttagcatatgttggttggttgagttaactgcttcatatttatttgctgtactggcaggttgacagggcaactgggaatcatgaagaaatagttcagcagaaccacgagactcagctcttaacaagcacttaataaatgttggttgaatgaataaatggctattgtagttattgaaaactaatacaattaaaggcaagtgagtttaaaaatcacagtcatttatataggtacctttctatttattcctaattaccaggaagcataataatgattaggtatttcaattatttttagtgaaaatttaatttgaataaaactaatagaacatcctatagataacagatcagtaatagcgacaaatttgttaaacgtgtgccagcaacagaaataattgtacaaagatccccattttacagatgcgatgacccagcttagaggggtcatctaattggtcttcccaattgtgaggttaggaattaaaagctggaattccaacacagctctatgctgtgctgttgcctctcagaaagatggctgggggttgagcagagagaatagctctcctggaacacattttcagaatataaactttttcagttatgatgtaatatatttatattattgtcattaagactatgatgaaaagacattagaggaagcaaaacaaagcctgatagttcagatatgagataagtaaagaagggtgtcaaatgacgaaatgctttttatgatgatatagaacgatgaaatgctcccttatgccaaaccttggcacagtacttctatgcccaccctggccactgattcagtcctactctcatatttgttcttcctgaagttggaaaataatgattcactggccatcctcagacattattacatgttgatctactgcagggttttattcaccctcctttaaaaacataaagtgaacattagccccaaataaagaacaccttgagacatcctgatgtcactgctatatctctattaggaaggagaaataaataacgttaagcatagagccatattttgtagggacttgctaaaaactgatttgttggtaaaactagtttatattgcaaatatacatatatatgtatatatatacatatattatatatatattttatattatatatatatatatacacacacacatacgtaaatatacacatcaacgatgatctctgtcatggtcagttggacttttcttccacagttaagggaagctcctcagatcttaccttcccaagcccacaaatgtatcccaatactggaaaaacagtgttggaaagaaaataaacttcatccaagaaaagatgttgatatggtttggatgttttgtcccc

SEQ ID NO: 14195 - RNA, 1020 nt, Homo sapiens
  source 1..1020: mol_type = other RNA
gctgggattacaggcatgagccaccgcgccaggctgaagtccatgattttaaaaactatttagtaaattttcattttgtagctcagttttgttagctatggttttataaataccctgataattacatttggtagcaaattagacacagtgtattaaagattgatgagacaaatatgttaaagataaaaattaattcaagagcacagatatgctatgcatactactaaaataaatacagtgatttataaatgagaaaaagttaacaatgaacagtgtttcagaagttgaaaaggtgacactaacagtgctaaatacacaggcttttatttgttttcttcagattgctttttcgtgaatataaagatgaggagtccattctgcaacctaaaaatatttacttattaaaactatattaatactttaataaactatacaaaaaggtaatgagacaaacatctgcatttatggaactgcatgtcagtcaggccagttccctgcagagggaattcccagcatgacctcattcatctgtgaggacacagagcagtccttgtttagacatacacattcatctactgctcatcatggtcagccttccacttcttgatggtttccttctgctatgaatgcgcatgtccggttgtctgcttcttagagcagacatttaccttcctcatccaccagccattggagggggactagggccacgcagatgattgattctacccattcttcggggagggtttcctggtggccctcttccatcatcatatctggaatcagatgagtttccatagcttcttctttttttcacatcttgctgaagcagagttttgaaaaacaaaaccacaaactcagctattccccagaagaaatctgttatcaaagataatctccatggagactgactccggctgtccaacacttgtccgttcgagatgtaaaccatcttgtcccacttccccgcttcggagccaccgggcgcctggcccctgtcggtttctgtatctccctctgctc

SEQ ID NO: 14196 - RNA, 4325 nt, Homo sapiens
  source 1..4325: mol_type = other RNA
gctgggattacaggcatgagccaccgcgcccagccaaaaagaagaaatattaagttgtccataatctgttatatctaactattataaagtataaataaaacaaaataagttttacattacttgtttctgtcacattgttcaaaattcttttgggcttaaagccaactatgaattttagttgagtaggaggacaatgggaaacagattctttttttgttgttattgaaatgtaagcaacttgcccttaaaatagtatgaatatccagttcaggtaacaactttcacttttaattagtcaaatatatattaaatataaaaatctaatgctgtacagatgtgactttggacattttaagtattagtttattcagaaacgcctttaaaaatcagtgtgtatagaactagctcatttcttaactgtcaaatttagaagtgcaacagtgggtcttcagagagaatatgcccaagaaaaactggataaaaagactgggtaaatacatcaaatgaaacagtgattcacttttgacaagactgaaatataagtatataatcactgatgcatatttattcagtaggcccatgtgattatgtggtttttaactaacagcatttatttttgcaaactgcttggcattcctccaagggaaaggagcttctagactacaaacactgagcacatacattttaaattaacacatgaattgcatatggattgttgatatgcttttagagtcttgtctctacagaagaaaaacacgttcctggggtccatgcctttttcagaggcacaatctatagcttggaacttaattgctgtccatggtatctggcctttaattataagaaattgttgacaccccaatacagggtgcatctaaatacataatgcaagaaaggaggttttagtggttaaacttcggcacgcttaaagattttaggaatgtaattatgccattaggcagtatttctttgtctatggacttaaaaagttttcttggggcattttaaagaggtttatcaaagttatattgttgaaaaactattttccctggaaataatgtcccctccttcccaccttctgccttgatattcttactggaaaaaaagtgaaattgttcagaattacaaccatatagggtttccaggcatagcatgggcacattgggaatggaagactagaagaccccagcaaggaatgtaggtacattaattgctgcctaccctgagaaataactctgagtttcttctcccaagtattcctcaaggatccattcattgtagagtcaacagatgtcttttagaattcattataataagaagtccatgaacatacacacactatccttgaatagttttacattatattttttctaggtagttcctgaatactttaatgagcttaataaatgagaaaatgtattgaaaggtctttgtaagttactatataaatatgacatgtgttttaataatatctgaatttggctgggaacaatggctcatgcctgtaatcctagcacttagggaggccaaggcgggaggatcccttgagctcaggagtttgagaccagcctgagcaaaatctctaaaaaaaaaatttctattagccaggtgtggtggcatgtgcctgtactgtagtctcagctacttgggaggtgagacaggaggatcactcgagcccaggagatggagactgcaatgagccatgattaagccactgcactccagcctaggtgacagagcagaccctgtctcaaaacaaaaaggaaaaaaagaatttctgaattttcatttttcatgaatgaaagtaaaaatcagagagaaaattttcacatatgacaatgtggattgtcatgtttaaagactctgaagttacgtagactatgagttatcatgttttcttttagcatgattctatacacctagctttaatttttgaagtctgatttaattgtgattttgacaatcagttactgaatgaggtagtccacattgcctagatatttgctgcatctggttactgattcacaaataattaagtagaatatatcacttatgtttttcctttatgtttaatagttctgtgaacattgacaatatattacttttagtggtacacagttcttgagaaaatgtcttgatttttacattgccatttgtgatatttttagcagtccaccacaatatcatttttataataaaaataaaatatactcattgatgatagagaaaatattgttaaagacctcttgggacaggaaaaggctcagtcataaaatcagatgcttattcattttcagctgtgtcattttgactcattactttcaagaataactataatattgctagacagttcattacactgagaagaactttccttgaacttcacatggagattgagtaaagctcttctatttgttttttgaagtactctctcagctcaggtctcttagcttttagtgttggtgtcagcaagccattttgaactgagaacatgtcagaatggatgtgaatggctttaacctgctcaaaagaatggagtccactttcttttcctaacctcaccatatcttccaaaatggctttcttcagatccttatttgtgcagagatctgcatatgttccttcaattcctctcttctgggcccaggagggcataacttcagggtcaggcacaacaatgcctaccaaaaaggcctttaagctgtccccatggacatagatttgcgccacaggttggctccggatgtagatgttctcaatcttctcgggtgcaacatattctccctgagcaagtttaaatatatgctttttccgatcaataattttaagagttcctgccggcagccattttccgatgtctccagtgtgaagccagccatcgctgtccagggcctccttcgtcctgtctggatctttcaagtagcctttgaacacatttggtcctctcacacatatctctccctctcctttgcaggcccagtagttcagttcctcaacatcaacgagcttgatatgattgcagggaagtggcgcccctacgtgccctgaggtccagtcgccaggagtggtgaaggtacatccagctgtgcactcagtttggccataaccttcataaacctggcaccctagagctgcccggagaaatcccagaactgttggtgatgctggggctgctccagtaacaatcatccgcacacacccaccaagactggcctgaatcttattaaagaagagttcatcccagatactatcattcctgatgattccactccggacctcggcttgcttacgctttgctgcaaactccaggagccagcgctttaatggtgtgtttgcctggctgaagatcttgtcgtacatccggttcagcagtcgtgggaccacagggaagatggtggggcatagagccttcatgtcatctgagagaaggcggatatctccctctgtcactttcagaaagcctgagaaatcagccaccacgttcccatgggtgagcatcgcaccttttgggttccctgtcgtgccgcttgtgaaacacacaatggagaggtcatcaggctgcgggggcacaggagcctggtgattctcttggccacagtcctccacggcctgcatggacttaatgaccaccccgcacttctgccctctctctttcagggcttcttcgaatgggtccatgaggatgatcagcttgaggcctggagtctccttcctctccacatgctctagcagaagcacagccttctgaggtttgtccacaatcacggtgctgatgtccgctgtattgatgatgtagcggatagccccagggcccagggtgtcatagagcgggaccaccaccatggaatatgtgtagcaggccagctccacaatgatccactctggccgattttgtgcaaaaacaccaataaactgatcagtgcatgctttacaattgtgctggagaagtccggaccccagaaattcagccctgtcggccacctcctggtaggacagccactggtaaggctgcttaggcttcctgaaaccaagacagggcccattccctgagatgctaagcccacggcggaacacctggtacatggtccgggcatcatcatagtagtgggtaagtagctgagggccagacccaatcacagatcgccgtgccccgccactgtcgagggtggtggccgagaggctgcggaaaaactgtcccaagtcacctagctcaggcagtcgcagtatcctcaggatctcctgtgtctgcatcttctccagaagtgagaggacaaacttccctgccctgcagcctggccggccgggtctggggcttgccccgcact

SEQ ID NO: 14197 - RNA, 4656 nt, Homo sapiens
  source 1..4656: mol_type = other RNA
gctgggattacaggcatgagccaccgcgcccagccaaaaagaagaaatattaagttgtccataatctgttatatctaactattataaagtataaataaaacaaaataagttttacattacttgtttctgtcacattgttcaaaattcttttgggcttaaagccaactatgaattttagttgagtaggaggacaatgggaaacagattctttttttgttgttattgaaatgtaagcaacttgcccttaaaatagtatgaatatccagttcaggtaacaactttcacttttaattagtcaaatatatattaaatataaaaatctaatgctgtacagatgtgactttggacattttaagtattagtttattcagaaacgcctttaaaaatcagtgtgtatagaactagctcatttcttaactgtcaaatttagaagtgcaacagtgggtcttcagagagaatatgcccaagaaaaactggataaaaagactgggtaaatacatcaaatgaaacagtgattcacttttgacaagactgaaatataagtatataatcactgatgcatatttattcagtaggcccatgtgattatgtggtttttaactaacagcatttatttttgcaaactgcttggcattcctccaagggaaaggagcttctagactacaaacactgagcacatacattttaaattaacacatgaattgcatatggattgttgatatgcttttagagtcttgtctctacagaagaaaaacacgttcctggggtccatgcctttttcagaggcacaatctatagcttggaacttaattgctgtccatggtatctggcctttaattataagaaattgttgacaccccaatacagggtgcatctaaatacataatgcaagaaaggaggttttagtggttaaacttcggcacgcttaaagattttaggaatgtaattatgccattaggcagtatttctttgtctatggacttaaaaagttttcttggggcattttaaagaggtttatcaaagttatattgttgaaaaactattttccctggaaataatgtcccctccttcccaccttctgccttgatattcttactggaaaaaaagtgaaattgttcagaattacaaccatatagggtttccaggcatagcatgggcacattgggaatggaagactagaagaccccagcaaggaatgtaggtacattaattgctgcctaccctgagaaataactctgagtttcttctcccaagtattcctcaaggatccattcattgtagagtcaacagatgtcttttagaattcattataataagaagtccatgaacatacacacactatccttgaatagttttacattatattttttctaggtagttcctgaatactttaatgagcttaataaatgagaaaatgtattgaaaggtctttgtaagttactatataaatatgacatgtgttttaataatatctgaatttggctgggaacaatggctcatgcctgtaatcctagcacttagggaggccaaggcgggaggatcccttgagctcaggagtttgagaccagcctgagcaaaatctctaaaaaaaaaatttctattagccaggtgtggtggcatgtgcctgtactgtagtctcagctacttgggaggtgagacaggaggatcactcgagcccaggagatggagactgcaatgagccatgattaagccactgcactccagcctaggtgacagagcagaccctgtctcaaaacaaaaaggaaaaaaagaatttctgaattttcatttttcatgaatgaaagtaaaaatcagagagaaaattttcacatatgacaatgtggattgtcatgtttaaagactctgaagttacgtagactatgagttatcatgttttcttttagcatgattctatacacctagctttaatttttgaagtctgatttaattgtgattttgacaatcagttactgaatgaggtagtccacattgcctagatatttgctgcatctggttactgattcacaaataattaagtagaatatatcacttatgtttttcctttatgtttaatagttctgtgaacattgacaatatattacttttagtggtacacagttcttgagaaaatgtcttgatttttacattgccatttgtgatatttttagcagtccaccacaatatcatttttataataaaaataaaatatactcattgatgatagagaaaatattgttaaagacctcttgggacaggaaaaggctcagtcataaaatcagatgcttattcattttcagctgtgtcattttgactcattactttcaagaataactataatattgctagacagttcattacactgagaagaactttccttgaacttcacatggagattgagtaaagctcttctatttgttttttgaagtactctctcagctcaggtctcttagcttttagtgttggtgtcagcaagccattttgaactgagaacatgtcagaatggatgtgaatggctttaacctgctcaaaagaatggagtccactttcttttcctaacctcaccatatcttccaaaatggctttcttcagatccttatttgtgcagagatctgcatatgttccttcaattcctctcttctgggcccaggagggcataacttcagggtcaggcacaacaatgcctaccaaaaaggcctttaagctgtccccatggacatagatttgcgccacaggttggctccggatgtagatgttctcaatcttctcgggtgcaacatattctccctgagcaagtttaaatatatgctttttccgatcaataattttaagagttcctgccggcagccattttccgatgtctccagtgtgaagccagccatcgctgtccagggcctccttcgtcctgtctggatctttcaagtagcctttgaacacatttggtcctctcacacatatctctccctctcctttgcaggcccagtagttcagttcctcaacatcaacgagcttgatatgattgcagggaagtggcgcccctacgtgccctgaggtccagtcgccaggagtggtgaaggtacatccagctgtgcactcagtttggccataaccttcataaacctggcaccctagagctgcccggagaaatcccagaactgttggtgatgctggggctgctccagtaacaatcatccgcacacacccaccaagactggcctgaatcttattaaagaagagttcatcccagatactatcattcctgatgattccactccggacctcggcttgcttacgctttgctgcaaactccaggagccagcgctttaatggtgtgtttgcctggctgaagatcttgtcgtacatccggttcagcagtcgtgggaccacagggaagatggtggggcatagagccttcatgtcatctgagagaaggcggatatctccctggaagaagccaacacgccctccgtggcaatagacgacagactgcaccattcgctcaaacatgtgtgctaaaggcaaataggaaatgtgcacatccgcacaagtgggagcccactgactctctgtcactttcagaaagcctgagaaatcagccaccacgttcccatgggtgagcatcgcaccttttgggttccctgtcgtgccgcttgtgaaacacacaatggagaggtcatcaggctgcgggggcacaggagcctggtgattctcttggccacagtcctccacggcctgcatggacttaatgaccaccccgcacttctgccctctctctttcagggcttcttcgaatgggtccatgaggatgatcagcttgaggcctggagtctccttcctctccacatgctctagcagaagcacagccttctgaggtttgtccacaatcacggtgctgatgtccgctgtattgatgatgtagcggatagccccagggcccagggtgtcatagagcgggaccaccaccatggaatatgtgtagcaggccagctccacaatgatccactctggccgattttgtgcaaaaacaccaataaactgatcagtgcatgctttacaattgtgctggagaagtccggaccccagaaattcagccctgtcggccacctcctggtaggacagccactggtaaggctgcttaggcttcctgaaaccaagacagggcccattccctgagatgctaagcccacggcggaacacctggtacatggtccgggcatcatcatagtagtgggtaagtagctgagggccagacccaatcacagatcgccgtgccccgccactgtcctctacttcttctgactgcatcaggaggttgcatggcggctgcaaggcctttggccggtgagtgaaccagtaggcaaggatggcagccagggcacccatactcacgagggtggtggccgagaggctgcggaaaaactgtcccaagtcacctagctcaggcagtcgcagtatcctcaggatctcctgtgtctgcatcttctccagaagtgagaggacaaactctacgaatagccagagggagccccccgacacgaggaagaaggtcagcatggcggtcagcggggcccggcccggcccggcccggcctccccgacccgcagccccgcagccccgcagcccagcagccccagcagtagccgcgccgccgccgccgct

SEQ ID NO: 14198 - RNA, 4550 nt, Homo sapiens
  source 1..4550: mol_type = other RNA
gctgggattacaggcatgagccaccgcgcccagccaaaaagaagaaatattaagttgtccataatctgttatatctaactattataaagtataaataaaacaaaataagttttacattacttgtttctgtcacattgttcaaaattcttttgggcttaaagccaactatgaattttagttgagtaggaggacaatgggaaacagattctttttttgttgttattgaaatgtaagcaacttgcccttaaaatagtatgaatatccagttcaggtaacaactttcacttttaattagtcaaatatatattaaatataaaaatctaatgctgtacagatgtgactttggacattttaagtattagtttattcagaaacgcctttaaaaatcagtgtgtatagaactagctcatttcttaactgtcaaatttagaagtgcaacagtgggtcttcagagagaatatgcccaagaaaaactggataaaaagactgggtaaatacatcaaatgaaacagtgattcacttttgacaagactgaaatataagtatataatcactgatgcatatttattcagtaggcccatgtgattatgtggtttttaactaacagcatttatttttgcaaactgcttggcattcctccaagggaaaggagcttctagactacaaacactgagcacatacattttaaattaacacatgaattgcatatggattgttgatatgcttttagagtcttgtctctacagaagaaaaacacgttcctggggtccatgcctttttcagaggcacaatctatagcttggaacttaattgctgtccatggtatctggcctttaattataagaaattgttgacaccccaatacagggtgcatctaaatacataatgcaagaaaggaggttttagtggttaaacttcggcacgcttaaagattttaggaatgtaattatgccattaggcagtatttctttgtctatggacttaaaaagttttcttggggcattttaaagaggtttatcaaagttatattgttgaaaaactattttccctggaaataatgtcccctccttcccaccttctgccttgatattcttactggaaaaaaagtgaaattgttcagaattacaaccatatagggtttccaggcatagcatgggcacattgggaatggaagactagaagaccccagcaaggaatgtaggtacattaattgctgcctaccctgagaaataactctgagtttcttctcccaagtattcctcaaggatccattcattgtagagtcaacagatgtcttttagaattcattataataagaagtccatgaacatacacacactatccttgaatagttttacattatattttttctaggtagttcctgaatactttaatgagcttaataaatgagaaaatgtattgaaaggtctttgtaagttactatataaatatgacatgtgttttaataatatctgaatttggctgggaacaatggctcatgcctgtaatcctagcacttagggaggccaaggcgggaggatcccttgagctcaggagtttgagaccagcctgagcaaaatctctaaaaaaaaaatttctattagccaggtgtggtggcatgtgcctgtactgtagtctcagctacttgggaggtgagacaggaggatcactcgagcccaggagatggagactgcaatgagccatgattaagccactgcactccagcctaggtgacagagcagaccctgtctcaaaacaaaaaggaaaaaaagaatttctgaattttcatttttcatgaatgaaagtaaaaatcagagagaaaattttcacatatgacaatgtggattgtcatgtttaaagactctgaagttacgtagactatgagttatcatgttttcttttagcatgattctatacacctagctttaatttttgaagtctgatttaattgtgattttgacaatcagttactgaatgaggtagtccacattgcctagatatttgctgcatctggttactgattcacaaataattaagtagaatatatcacttatgtttttcctttatgtttaatagttctgtgaacattgacaatatattacttttagtggtacacagttcttgagaaaatgtcttgatttttacattgccatttgtgatatttttagcagtccaccacaatatcatttttataataaaaataaaatatactcattgatgatagagaaaatattgttaaagacctcttgggacaggaaaaggctcagtcataaaatcagatgcttattcattttcagctgtgtcattttgactcattactttcaagaataactataatattgctagacagttcattacactgagaagaactttccttgaacttcacatggagattgagtaaagctcttctatttgttttttgaagtactctctcagctcaggtctcttagcttttagtgttggtgtcagcaagccattttgaactgagaacatgtcagaatggatgtgaatggctttaacctgctcaaaagaatggagtccactttcttttcctaacctcaccatatcttccaaaatggctttcttcagatccttatttgtgcagagatctgcatatgttccttcaattcctctcttctgggcccaggagggcataacttcagggtcaggcacaacaatgcctaccaaaaaggcctttaagctgtccccatggacatagatttgcgccacaggttggctccggatgtagatgttctcaatcttctcgggtgcaacatattctccctgagcaagtttaaatatatgctttttccgatcaataattttaagagttcctgccggcagccattttccgatgtctccagtgtgaagccagccatcgctgtccagggcctccttcgtcctgtctggatctttcaagtagcctttgaacacatttggtcctctcacacatatctctccctctcctttgcaggcccagtagttcagttcctcaacatcaacgagcttgatatgattgcagggaagtggcgcccctacgtgccctgaggtccagtcgccaggagtggtgaaggtacatccagctgtgcactcagtttggccataaccttcataaacctggcaccctagagctgcccggagaaatcccagaactgttggtgatgctggggctgctccagtaacaatcatccgcacacacccaccaagactggcctgaatcttattaaagaagagttcatcccagatactatcattcctgatgattccactccggacctcggcttgcttacgctttgctgcaaactccaggagccagcgctttaatggtgtgtttgcctggctgaagatcttgtcgtacatccggttcagcagtcgtgggaccacagggaagatggtggggcatagagccttcatgtcatctgagagaaggcggatatctccctggaagaagccaacacgccctccgtggcaatagacgacagactgcaccattcgctcaaacatgtgtgctaaaggcaaataggaaatgtgcacatccgcacaagtgggagcccactgactctctgtcactttcagaaagcctgagaaatcagccaccacgttcccatgggtgagcatcgcaccttttgggttccctgtcgtgccgcttgtgaaacacacaatggagaggtcatcaggctgcgggggcacaggagcctggtgattctcttggccacagtcctccacggcctgcatggacttaatgaccaccccgcacttctgccctctctctttcagggcttcttcgaatgggtccatgaggatgatcagcttgaggcctggagtctccttcctctccacatgctctagcagaagcacagccttctgaggtttgtccacaatcacggtgctgatgtccgctgtattgatgatgtagcggatagccccagggcccagggtgtcatagagcgggaccaccaccatggaatatgtgtagcaggccagctccacaatgatccactctggccgattttgtgcaaaaacaccaataaactgatcagtgcatgctttacaattgtgctggagaagtccggaccccagaaattcagccctgtcggccacctcctggtaggacagccactggtaaggctgcttaggcttcctgaaaccaagacagggcccattccctgagatgctaagcccacggcggaacacctggtacatggtccgggcatcatcatagtagtgggtaagtagctgagggccagacccaatcacagatcgccgtgccccgccactgtcctctacttcttctgactgcatcaggaggttgcatggcggctgcaaggcctttggccggtgagtgaaccagtaggcaaggatggcagccagggcacccatactcacgagggtggtggccgagaggctgcggaaaaactgtcccaagtcacctagctcaggcagtcgcagtatcctcaggatctcctgtgtctgcatcttctccagaagtgagaggacaaacttccctgccctgcagcctggccggccgggtctggggcttgccccgcact

SEQ ID NO: 14199 - RNA, 4551 nt, Homo sapiens
  source 1..4551: mol_type = other RNA
gctgggattacaggcatgagccaccgcgcccagccaaaaagaagaaatattaagttgtccataatctgttatatctaactattataaagtataaataaaacaaaataagttttacattacttgtttctgtcacattgttcaaaattcttttgggcttaaagccaactatgaattttagttgagtaggaggacaatgggaaacagattctttttttgttgttattgaaatgtaagcaacttgcccttaaaatagtatgaatatccagttcaggtaacaactttcacttttaattagtcaaatatatattaaatataaaaatctaatgctgtacagatgtgactttggacattttaagtattagtttattcagaaacgcctttaaaaatcagtgtgtatagaactagctcatttcttaactgtcaaatttagaagtgcaacagtgggtcttcagagagaatatgcccaagaaaaactggataaaaagactgggtaaatacatcaaatgaaacagtgattcacttttgacaagactgaaatataagtatataatcactgatgcatatttattcagtaggcccatgtgattatgtggtttttaactaacagcatttatttttgcaaactgcttggcattcctccaagggaaaggagcttctagactacaaacactgagcacatacattttaaattaacacatgaattgcatatggattgttgatatgcttttagagtcttgtctctacagaagaaaaacacgttcctggggtccatgcctttttcagaggcacaatctatagcttggaacttaattgctgtccatggtatctggcctttaattataagaaattgttgacaccccaatacagggtgcatctaaatacataatgcaagaaaggaggttttagtggttaaacttcggcacgcttaaagattttaggaatgtaattatgccattaggcagtatttctttgtctatggacttaaaaagttttcttggggcattttaaagaggtttatcaaagttatattgttgaaaaactattttccctggaaataatgtcccctccttcccaccttctgccttgatattcttactggaaaaaaagtgaaattgttcagaattacaaccatatagggtttccaggcatagcatgggcacattgggaatggaagactagaagaccccagcaaggaatgtaggtacattaattgctgcctaccctgagaaataactctgagtttcttctcccaagtattcctcaaggatccattcattgtagagtcaacagatgtcttttagaattcattataataagaagtccatgaacatacacacactatccttgaatagttttacattatattttttctaggtagttcctgaatactttaatgagcttaataaatgagaaaatgtattgaaaggtctttgtaagttactatataaatatgacatgtgttttaataatatctgaatttggctgggaacaatggctcatgcctgtaatcctagcacttagggaggccaaggcgggaggatcccttgagctcaggagtttgagaccagcctgagcaaaatctctaaaaaaaaaatttctattagccaggtgtggtggcatgtgcctgtactgtagtctcagctacttgggaggtgagacaggaggatcactcgagcccaggagatggagactgcaatgagccatgattaagccactgcactccagcctaggtgacagagcagaccctgtctcaaaacaaaaaggaaaaaaagaatttctgaattttcatttttcatgaatgaaagtaaaaatcagagagaaaattttcacatatgacaatgtggattgtcatgtttaaagactctgaagttacgtagactatgagttatcatgttttcttttagcatgattctatacacctagctttaatttttgaagtctgatttaattgtgattttgacaatcagttactgaatgaggtagtccacattgcctagatatttgctgcatctggttactgattcacaaataattaagtagaatatatcacttatgtttttcctttatgtttaatagttctgtgaacattgacaatatattacttttagtggtacacagttcttgagaaaatgtcttgatttttacattgccatttgtgatatttttagcagtccaccacaatatcatttttataataaaaataaaatatactcattgatgatagagaaaatattgttaaagacctcttgggacaggaaaaggctcagtcataaaatcagatgcttattcattttcagctgtgtcattttgactcattactttcaagaataactataatattgctagacagttcattacactgagaagaactttccttgaacttcacatggagattgagtaaagctcttctatttgttttttgaagtactctctcagctcaggtctcttagcttttagtgttggtgtcagcaagccattttgaactgagaacatgtcagaatggatgtgaatggctttaacctgctcaaaagaatggagtccactttcttttcctaacctcaccatatcttccaaaatggctttcttcagatccttatttgtgcagagatctgcatatgttccttcaattcctctcttctgggcccaggagggcataacttcagggtcaggcacaacaatgcctaccaaaaaggcctttaagctgtccccatggacatagatttgcgccacaggttggctccggatgtagatgttctcaatcttctcgggtgcaacatattctccctgagcaagtttaaatatatgctttttccgatcaataattttaagagttcctgccggcagccattttccgatgtctccagtgtgaagccagccatcgctgtccagggcctccttcgtcctgtctggatctttcaagtagcctttgaacacatttggtcctctcacacatatctctccctctcctttgcaggcccagtagttcagttcctcaacatcaacgagcttgatatgattgcagggaagtggcgcccctacgtgccctgaggtccagtcgccaggagtggtgaaggtacatccagctgtgcactcagtttggccataaccttcataaacctggcaccctagagctgcccggagaaatcccagaactgttggtgatgctggggctgctccagtaacaatcatccgcacacacccaccaagactggcctgaatcttattaaagaagagttcatcccagatactatcattcctgatgattccactccggacctcggcttgcttacgctttgctgcaaactccaggagccagcgctttaatggtgtgtttgcctggctgaagatcttgtcgtacatccggttcagcagtcgtgggaccacagggaagatggtggggcatagagccttcatgtcatctgagagaaggcggatatctccctggaagaagccaacacgccctccgtggcaatagacgacagactgcaccattcgctcaaacatgtgtgctaaaggcaaataggaaatgtgcacatccgcacaagtgggagcccactgactctctgtcactttcagaaagcctgagaaatcagccaccacgttcccatgggtgagcatcgcaccttttgggttccctgtcgtgccgcttgtgaaacacacaatggagaggtcatcaggctgcgggggcacaggagcctggtgattctcttggccacagtcctccacggcctgcatggacttaatgaccaccccgcacttctgccctctctctttcagggcttcttcgaatgggtccatgaggatgatcagcttgaggcctggagtctccttcctctccacatgctctagcagaagcacagccttctgaggtttgtccacaatcacggtgctgatgtccgctgtattgatgatgtagcggatagccccagggcccagggtgtcatagagcgggaccaccaccatggaatatgtgtagcaggccagctccacaatgatccactctggccgattttgtgcaaaaacaccaataaactgatcagtgcatgctttacaattgtgctggagaagtccggaccccagaaattcagccctgtcggccacctcctggtaggacagccactggtaaggctgcttaggcttcctgaaaccaagacagggcccattccctgagatgctaagcccacggcggaacacctggtacatggtccgggcatcatcatagtagtgggtaagtagctgagggccagacccaatcacagatcgccgtgccccgccactgtcgagggtggtggccgagaggctgcggaaaaactgtcccaagtcacctagctcaggcagtcgcagtatcctcaggatctcctgtgtctgcatcttctccagaagtgagaggacaaactctacgaatagccagagggagccccccgacacgaggaagaaggtcagcatggcggtcagcggggcccggcccggcccggcccggcctccccgacccgcagccccgcagccccgcagcccagcagccccagcagtagccgcgccgccgccgccgct

SEQ ID NO: 14200 - RNA, 4656 nt, Homo sapiens
  source 1..4656: mol_type = other RNA
gctgggattacaggcatgagccaccgcgcccagccaaaaagaagaaatattaagttgtccataatctgttatatctaactattataaagtataaataaaacaaaataagttttacattacttgtttctgtcacattgttcaaaattcttttgggcttaaagccaactatgaattttagttgagtaggaggacaatgggaaacagattctttttttgttgttattgaaatgtaagcaacttgcccttaaaatagtatgaatatccagttcaggtaacaactttcacttttaattagtcaaatatatattaaatataaaaatctaatgctgtacagatgtgactttggacattttaagtattagtttattcagaaacgcctttaaaaatcagtgtgtatagaactagctcatttcttaactgtcaaatttagaagtgcaacagtgggtcttcagagagaatatgcccaagaaaaactggataaaaagactgggtaaatacatcaaatgaaacagtgattcacttttgacaagactgaaatataagtatataatcactgatgcatatttattcagtaggcccatgtgattatgtggtttttaactaacagcatttatttttgcaaactgcttggcattcctccaagggaaaggagcttctagactacaaacactgagcacatacattttaaattaacacatgaattgcatatggattgttgatatgcttttagagtcttgtctctacagaagaaaaacacgttcctggggtccatgcctttttcagaggcacaatctatagcttggaacttaattgctgtccatggtatctggcctttaattataagaaattgttgacaccccaatacagggtgcatctaaatacataatgcaagaaaggaggttttagtggttaaacttcggcacgcttaaagattttaggaatgtaattatgccattaggcagtatttctttgtctatggacttaaaaagttttcttggggcattttaaagaggtttatcaaagttatattgttgaaaaactattttccctggaaataatgtcccctccttcccaccttctgccttgatattcttactggaaaaaaagtgaaattgttcagaattacaaccatatagggtttccaggcatagcatgggcacattgggaatggaagactagaagaccccagcaaggaatgtaggtacattaattgctgcctaccctgagaaataactctgagtttcttctcccaagtattcctcaaggatccattcattgtagagtcaacagatgtcttttagaattcattataataagaagtccatgaacatacacacactatccttgaatagttttacattatattttttctaggtagttcctgaatactttaatgagcttaataaatgagaaaatgtattgaaaggtctttgtaagttactatataaatatgacatgtgttttaataatatctgaatttggctgggaacaatggctcatgcctgtaatcctagcacttagggaggccaaggcgggaggatcccttgagctcaggagtttgagaccagcctgagcaaaatctctaaaaaaaaaatttctattagccaggtgtggtggcatgtgcctgtactgtagtctcagctacttgggaggtgagacaggaggatcactcgagcccaggagatggagactgcaatgagccatgattaagccactgcactccagcctaggtgacagagcagaccctgtctcaaaacaaaaaggaaaaaaagaatttctgaattttcatttttcatgaatgaaagtaaaaatcagagagaaaattttcacatatgacaatgtggattgtcatgtttaaagactctgaagttacgtagactatgagttatcatgttttcttttagcatgattctatacacctagctttaatttttgaagtctgatttaattgtgattttgacaatcagttactgaatgaggtagtccacattgcctagatatttgctgcatctggttactgattcacaaataattaagtagaatatatcacttatgtttttcctttatgtttaatagttctgtgaacattgacaatatattacttttagtggtacacagttcttgagaaaatgtcttgatttttacattgccatttgtgatatttttagcagtccaccacaatatcatttttataataaaaataaaatatactcattgatgatagagaaaatattgttaaagacctcttgggacaggaaaaggctcagtcataaaatcagatgcttattcattttcagctgtgtcattttgactcattactttcaagaataactataatattgctagacagttcattacactgagaagaactttccttgaacttcacatggagattgagtaaagctcttctatttgttttttgaagtactctctcagctcaggtctcttagcttttagtgttggtgtcagcaagccattttgaactgagaacatgtcagaatggatgtgaatggctttaacctgctcaaaagaatggagtccactttcttttcctaacctcaccatatcttccaaaatggctttcttcagatccttatttgtgcagagatctgcatatgttccttcaattcctctcttctgggcccaggagggcataacttcagggtcaggcacaacaatgcctaccaaaaaggcctttaagctgtccccatggacatagatttgcgccacaggttggctccggatgtagatgttctcaatcttctcgggtgcaacatattctccctgagcaagtttaaatatatgctttttccgatcaataattttaagagttcctgccggcagccattttccgatgtctccagtgtgaagccagccatcgctgtccagggcctccttcgtcctgtctggatctttcaagtagcctttgaacacatttggtcctctcacacatatctctccctctcctttgcaggcccagtagttcagttcctcaacatcaacgagcttgatatgattgcagggaagtggcgcccctacgtgccctgaggtccagtcgccaggagtggtgaaggtacatccagctgtgcactcagtttggccataaccttcataaacctggcaccctagagctgcccggagaaatcccagaactgttggtgatgctggggctgctccagtaacaatcatccgcacacacccaccaagactggcctgaatcttattaaagaagagttcatcccagatactatcattcctgatgattccactccggacctcggcttgcttacgctttgctgcaaactccaggagccagcgctttaatggtgtgtttgcctggctgaagatcttgtcgtacatccggttcagcagtcgtgggaccacagggaagatggtggggcatagagccttcatgtcatctgagagaaggcggatatctccctggaagaagccaacacgccctccgtggcaatagacgacagactggattactctctcaaacatgtgagccagaggcaggaaggagatgagcacatcgtcctgtctcggaaagatcactttctctgtcactttcagaaagcctgagaaatcagccaccacgttcccatgggtgagcatcgcaccttttgggttccctgtcgtgccgcttgtgaaacacacaatggagaggtcatcaggctgcgggggcacaggagcctggtgattctcttggccacagtcctccacggcctgcatggacttaatgaccaccccgcacttctgccctctctctttcagggcttcttcgaatgggtccatgaggatgatcagcttgaggcctggagtctccttcctctccacatgctctagcagaagcacagccttctgaggtttgtccacaatcacggtgctgatgtccgctgtattgatgatgtagcggatagccccagggcccagggtgtcatagagcgggaccaccaccatggaatatgtgtagcaggccagctccacaatgatccactctggccgattttgtgcaaaaacaccaataaactgatcagtgcatgctttacaattgtgctggagaagtccggaccccagaaattcagccctgtcggccacctcctggtaggacagccactggtaaggctgcttaggcttcctgaaaccaagacagggcccattccctgagatgctaagcccacggcggaacacctggtacatggtccgggcatcatcatagtagtgggtaagtagctgagggccagacccaatcacagatcgccgtgccccgccactgtcctctacttcttctgactgcatcaggaggttgcatggcggctgcaaggcctttggccggtgagtgaaccagtaggcaaggatggcagccagggcacccatactcacgagggtggtggccgagaggctgcggaaaaactgtcccaagtcacctagctcaggcagtcgcagtatcctcaggatctcctgtgtctgcatcttctccagaagtgagaggacaaactctacgaatagccagagggagccccccgacacgaggaagaaggtcagcatggcggtcagcggggcccggcccggcccggcccggcctccccgacccgcagccccgcagccccgcagcccagcagccccagcagtagccgcgccgccgccgccgct

SEQ ID NO: 14201 - RNA, 4657 nt, Homo sapiens
  source 1..4657: mol_type = other RNA
gctgggattacaggcatgagccaccgcgcccagccaaaaagaagaaatattaagttgtccataatctgttatatctaactattataaagtataaataaaacaaaataagttttacattacttgtttctgtcacattgttcaaaattcttttgggcttaaagccaactatgaattttagttgagtaggaggacaatgggaaacagattctttttttgttgttattgaaatgtaagcaacttgcccttaaaatagtatgaatatccagttcaggtaacaactttcacttttaattagtcaaatatatattaaatataaaaatctaatgctgtacagatgtgactttggacattttaagtattagtttattcagaaacgcctttaaaaatcagtgtgtatagaactagctcatttcttaactgtcaaatttagaagtgcaacagtgggtcttcagagagaatatgcccaagaaaaactggataaaaagactgggtaaatacatcaaatgaaacagtgattcacttttgacaagactgaaatataagtatataatcactgatgcatatttattcagtaggcccatgtgattatgtggtttttaactaacagcatttatttttgcaaactgcttggcattcctccaagggaaaggagcttctagactacaaacactgagcacatacattttaaattaacacatgaattgcatatggattgttgatatgcttttagagtcttgtctctacagaagaaaaacacgttcctggggtccatgcctttttcagaggcacaatctatagcttggaacttaattgctgtccatggtatctggcctttaattataagaaattgttgacaccccaatacagggtgcatctaaatacataatgcaagaaaggaggttttagtggttaaacttcggcacgcttaaagattttaggaatgtaattatgccattaggcagtatttctttgtctatggacttaaaaagttttcttggggcattttaaagaggtttatcaaagttatattgttgaaaaactattttccctggaaataatgtcccctccttcccaccttctgccttgatattcttactggaaaaaaagtgaaattgttcagaattacaaccatatagggtttccaggcatagcatgggcacattgggaatggaagactagaagaccccagcaaggaatgtaggtacattaattgctgcctaccctgagaaataactctgagtttcttctcccaagtattcctcaaggatccattcattgtagagtcaacagatgtcttttagaattcattataataagaagtccatgaacatacacacactatccttgaatagttttacattatattttttctaggtagttcctgaatactttaatgagcttaataaatgagaaaatgtattgaaaggtctttgtaagttactatataaatatgacatgtgttttaataatatctgaatttggctgggaacaatggctcatgcctgtaatcctagcacttagggaggccaaggcgggaggatcccttgagctcaggagtttgagaccagcctgagcaaaatctctaaaaaaaaaatttctattagccaggtgtggtggcatgtgcctgtactgtagtctcagctacttgggaggtgagacaggaggatcactcgagcccaggagatggagactgcaatgagccatgattaagccactgcactccagcctaggtgacagagcagaccctgtctcaaaacaaaaaggaaaaaaagaatttctgaattttcatttttcatgaatgaaagtaaaaatcagagagaaaattttcacatatgacaatgtggattgtcatgtttaaagactctgaagttacgtagactatgagttatcatgttttcttttagcatgattctatacacctagctttaatttttgaagtctgatttaattgtgattttgacaatcagttactgaatgaggtagtccacattgcctagatatttgctgcatctggttactgattcacaaataattaagtagaatatatcacttatgtttttcctttatgtttaatagttctgtgaacattgacaatatattacttttagtggtacacagttcttgagaaaatgtcttgatttttacattgccatttgtgatatttttagcagtccaccacaatatcatttttataataaaaataaaatatactcattgatgatagagaaaatattgttaaagacctcttgggacaggaaaaggctcagtcataaaatcagatgcttattcattttcagctgtgtcattttgactcattactttcaagaataactataatattgctagacagttcattacactgagaagaactttccttgaacttcacatggagattgagtaaagctcttctatttgttttttgaagtactctctcagctcaggtctcttagcttttagtgttggtgtcagcaagccattttgaactgagaacatgtcagaatggatgtgaatggctttaacctgctcaaaagaatggagtccactttcttttcctaacctcaccatatcttccaaaatggctttcttcagatccttatttgtgcagagatctgcatatgttccttcaattcctctcttctgggcccaggagggcataacttcagggtcaggcacaacaatgcctaccaaaaaggcctttaagctgtccccatggacatagatttgcgccacaggttggctccggatgtagatgttctcaatcttctcgggtgcaacatattctccctgagcaagtttaaatatatgctttttccgatcaataattttaagagttcctgccggcagccattttccgatgtctccagtgtgaagccagccatcgctgtccagggcctccttcgtcctgtctggatctttcaagtagcctttgaacacatttggtcctctcacacatatctctccctctcctttgcaggcccagtagttcagttcctcaacatcaacgagcttgatatgattgcagggaagtggcgcccctacgtgccctgaggtccagtcgccaggagtggtgaaggtacatccagctgtgcactcagtttggccataaccttcataaacctggcaccctagagctgcccggagaaatcccagaactgttggtgatgctggggctgctccagtaacaatcatccgcacacacccaccaagactggcctgaatcttattaaagaagagttcatcccagatactatcattcctgatgattccactccggacctcggcttgcttacgctttgctgcaaactccaggagccagcgctttaatggtgtgtttgcctggctgaagatcttgtcgtacatccggttcagcagtcgtgggaccacagggaagatggtggggcatagagccttcatgtcatctgagagaaggcggatatctccctggaagaagccaacacgccctccgtggcaatagacgacagactggattactctctcaaacatgtgagccagaggcaggaaggagatgagcacatcgtcctgtctcggaaagatcactttctctgtcactttcagaaagcctgagaaatcagccaccacgttcccatgggtgagcatcgcaccttttgggttccctgtcgtgccgcttgtgaaacacacaatggagaggtcatcaggctgcgggggcacaggagcctggtgattctcttggccacagtcctccacggcctgcatggacttaatgaccaccccgcacttctgccctctctctttcagggcttcttcgaatgggtccatgaggatgatcagcttgaggcctggagtctccttcctctccacatgctctagcagaagcacagccttctgaggtttgtccacaatcacggtgctgatgtccgctgtattgatgatgtagcggatagccccagggcccagggtgtcatagagcgggaccaccaccatggaatatgtgtagcaggccagctccacaatgatccactctggccgattttgtgcaaaaacaccaataaactgatcagtgcatgctttacaattgtgctggagaagtccggaccccagaaattcagccctgtcggccacctcctggtaggacagccactggtaaggctgcttaggcttcctgaaaccaagacagggcccattccctgagatgctaagcccacggcggaacacctggtacatggtccgggcatcatcatagtagtgggtaagtagctgagggccagacccaatcacagatcgccgtgccccgccactgtcctctacttcttctgactgcatcaggaggttgcatggcggctgcaaggcctttggccggtgagtgaaccagtaggcaaggatggcagccagggcacccatactcacgagggtggtggccgagaggctgcggaaaaactgtcccaagtcacctagctcaggcagtcgcagtatcctcaggatctcctgtgtctgcatcttctccagaagtgagaggacaaactctggcattctgcggaaaccggctggaagggggagcacgggcgacgagcgccagagcgtgacattgagcccaccccgccgccacccaccccatcaacacgcgaccctgcccccgcgcgactcgcagcctgggttttatggctgggcaggctcgaat

SEQ ID NO: 14202 - RNA, 478 nt, Homo sapiens
  source 1..478: mol_type = other RNA
gctgggattacaggcatgagccaccgcgcccagccaaataatatagaatgttattcctctctcatgcaacactacaaaacaggaaggacgtcctcagctccatgaagttctccagggaccctggaactcctcccctgccttacagcttccatccttgtgtctaagattgttgctccggttgtcctcttcttggtcacagctggctaccagcaccatattggagttccaaccaggtctgggcttttgtccccatgtctgttctcacggcggaatgtagatctgctgcaatgtcggcctaacactggccacagtctcgccatttccattttcccttgctcctcatcatccatcttaatgctattgctcttggtttcacatggttttagtccacaccatatgataactcacatttgtttaaatccagtgtcttttgtgtgctcatgacacatttccaaattcctgaaaatttggttgtgca

SEQ ID NO: 14203 - RNA, 264 nt, Homo sapiens
  source 1..264: mol_type = other RNA
gctgggattacaggcatgagccaccgcgcccagccaaataatatagaatgttattcctctctcatgcaacactacaaaacaggaaggacgtcctcagctccatgaagttctccagggaccctggaactcctcccctgccttacagcttccatccttgtgtctaagattgttgctccggttgtcctcttcttggtcacagctggctaccagcaccatattggagttccaacccttataaaagaggccagagagaaaccctttgcc

SEQ ID NO: 14204 - RNA, 2119 nt, Homo sapiens
  source 1..2119: mol_type = other RNA
gctgggattacaggcatgagccaccgcgcccagccaagagtctgcttttagctttcctgtcttagtgcccctgaaggaaagggaatgtgcttgttccttattattaaggcccactgttttactggggcccatcgtatgagggtgaagtttggcagttacccaagatactttccccccacctccctttgtgtcccagctgtcttatccgtgttttactgtctgctctttctggctgcttgtagttagaagagaagtgatttccttgaaatgcatgaggctagaaagggagctggaatttaaagtggcggtgtttgtctgagatgacagtactcctgctctatcattccagaccctatggttataaaaggacaagaggggacatgttctttctagctacttcctgctgatgcgggggtggagagttttttggtcttagattgactgtaggatcaacaccatttgtagatgtttttgggtagttgcgaaatggccatgattctgtcggttaaaaatttttgataaaggttaattaggcagagtaaaaacattagtcctaggcttttcagcagcattttttattaggcccgactggttgagacagaagtaactttttttttttttttttttaatgacaggcagaggtgcatgtttggaaagacccatgtgttattttttgttagtaactgttattcctgctatgaggataataattaagcaaaatgctacagtaattgagattctctgtcagatattccactctgagggttcacagtcctactgcaaatagtagagtgagtacagcagttcccgcgagggtgtcatagtaaataattttcattaaaaaaggttttaatagttggcttaaaaggagaagtagaaacgacaaaaagtatttggtgaggtggggttgagactgagtaagatgagcaatttttacttagttacttaacttttatgatttttagcttaagatttcttatttatttttttacatgaataggactttttttggactgttaggggttgctttctcagctctttaggctttgacttgaatatgatgtatccaggagttgatttctgtaacggatataatttaaacacacatcagaaaccctgtacagggactgtgcacacaaaatatgaggccagttttccaagggtttcattggcttcttaagtttgattccttagaggagagcacaccattccagtcaaagccttgggaaaataaccagtttttccaattgtattccatcaggggagagaccatgatcacaaaggtggttttcccagggcgagtcttctccattgtactctggatgtgctgatccctgcaatttccccaaaggtgggaaactcgacttcataatttgtggtaatggggaactgcatttgcactctcccctggcattttgtaaaagaaaagaaaaaaacacagagagtactaagcgcaccctgagagtttcggattcagaatgaggtggaaaagtcagaattaggtgaaattgttaacctgggacaagttcctgggagatactggcatctcttgtactaggaaaagcacgttttgagaatcatgggtctgggtcactgcctttgagctgggaacctcagcagacaggatgcaggggcctcagcttggatgaacagaccctctaggaacactgactggtccttctcaggcctgatggagacagactgtggggcagggcttaaggatagagggccaggattaggaaagggggcttgtaggcctggccaggcacagaggtgtagtttgttaaggaaagccagtctccctcagtggggaagctgcagcctggccctagaatcaactccaacactcaacacccaatgccagccaggcttcagtcttggacctgaccacaagtgacccatgacataccctgaccccaccacagcctgggtcctacacccagccactaagtgaccactgaccccagctgctgaccctggacccagaccaggcctggctgggactcctacttggccttgatctcagatgtcctgaagcagtatttcattggtcactgtgggacagcttttgcaagtgcagtccaatctgctgacatcacatcccaccctctctcaaaac

SEQ ID NO: 14205 - RNA, 3555 nt, Homo sapiens
  source 1..3555: mol_type = other RNA
gctgggattacaggcatgagccaccgcgcccagccactattttttaagttagtagcacacttaacatataaccaaccttaagttagaaaagtcattttttgaaggcacagtttgtttccagctcaactgtggaaatcaaaatctgtctgcagtaccaaatcccatcccacagtcagcccagccctggcaccattttgcttgtctccatgaaatgtgtctagtctagagggtagcatttttttgtcgatcccaatcatcatgtgaaaagtttctggagccatgttacgtcttccttcattctctgtgaaaatgcaagcaactcatttataaagtagcatcagcaaccaggccttcctgggcatgggagtggggaagaagtggcagaaaggaccagctcgctgtcctgtagcttacggacagtcccctcagcacaggacgtagaacgagagggtctgaacaagaacaggacaaaacgaggccctctaatatgtcagacgaagacaaatttccagaaaagtgaaggcaactccccttccatatacctggggttaagaaaaaaaaaaccaaaaaacagagaagggcgggtgactggcttcatcagtccagcaaaagacagggaatgtgcataaaataagatgttactgtgcttcaagtcagttgaatcactaatctcattaggcaagtggaagtctgctgagaatgtggcagtggcctttacatgtatttattttaaataattagcttaggtctgagctataatgactaatctccacgagtctatgcctgacggtgataaaaagttgacatacatggaaggtgttagaggaaagaaccagaaacaattacagtaagtggaaccgtgcacaaaagctgctctgcatcccgggttcatgcttttaagcagcctttttgctgaaagcctcacgaagtagttttgtttgggttgagtgttatgtttaaaatttcccttctaccagttattgagaaaataataatgccgagctcatctaataaacaaatgtctagttcgataagctttaatcaggccctcacaccctgggatggtcgttaatgacatggatcagaatccctgaggtggctggaatctaacaagtgggtagcacagaaagctcaccttgcctatggaggctgtggatatttttaggaaggtcatgcattatgggatgggaatttttataaacaaattgctacataaaaactaatgcactgttgcagcacttgtggaggtttcctttgctttgagacaccactgtttataggctgcagactgtaaagggaagtactgggaaatggcaaaggtcacatgggccagtgccatgttttaaggtcaaaggcactgttattttaagtgacctatctcattattaaaatcagtcactttcaccatcttcaaaatattttgtttttttaaaaagacaagggccttgtggctccaactattttgttggatgtaccaacataaataaatcagttttaattgatgcttctgcatgatttcttttgtaaaatgaaaggagaaaatgaactgggccagttaaaatggtatctgggctttttgcccccttagcaaaatccttctatacaaagtcagcgtcatttatagagtgccagtcctaaaaccaggtggcagagaaataagtgatgattcaagttaccttgcaagaagtgcagaagagtgggtgggaatgctagacaggtcaggagacccccggtaccaaataaacattttgccctactgaggcctgcctaatggtgattcccagaggggtggaggaagaccattgtgcagctgcatctgtgcaatactccattcccacaaactctattgggcgcccctgtcggtcagcctcgcagcctcgagccagtggaagacctgttgcaaatcacagatggagagttacagatgggagcacgtggggaagaggggctcacccaattccccacacatttccaggagtcgcagtgagcagtgctggtgtgaagccctcctactaatatacatgccaaggatggggggctggagggaagcggggacatctgccaacaaaagagcaagatggcacactctatttcccattctaacactgatcctttctgggaggatgaaagaatcacagataatgtgctcagagagtgtgtgtgtgtgtgtgtgtgtgtgtgtgtgtgtgtgtgtgtgtgaatgatgactcctaaacaaaggtgtgggaaggaccctcctccaccaaacgactggttcacaggcccccttaacactctgactcatggtaaggcttaggaatgagaaatagaggctcatggctgcaagactgaaattctgttcccatctttccatatgctcattaaaatgagaaatgcaactcttcttattccagcatggtaatcaaacgcccaagatatgcagggccaggctactgtgctcagacaaaaactctaataagcattttgctggaagaacttggtgaggtgttaaccctaggaaaatgtgggacaaacacttccttataacagcaaaaatgtcttaagacctactctattataacatttgcaaacacacattaatttacatactaaaatagtaaatgaaatttcttggaagttcaaaaaaagatctttcaaatcttttcatcacaatagagtggaaatccgtctgtcttcagagttgtcgaacttttctttctgtgctttttatgttgacatctaacttgtccactttggttgtcagccggtcaagaatgtcatcttgctcctcaatttctgtctgcatccccagggctatgtccttcagacgacccagtcccatggacagctcatctaggttgctgtcgatcttctggtgataggctcgaaggtgtgggttctttgggtaagcatcagtactcatggcagaaccagcccctctggggacagggtctgtatcatccagctttctaaggtttgggtggctggcctggtactttgcttcctgttctttacttgtacttatagcttctttcaatctgttgttgggctgggaggtgagggtgccattctgttcaggtggggtctctactggtttggatttgaagtaattgaccagccccccaaacacgctcttaatgctattgatgtgtttctggctgatcttcaaatcttggtccatcttgtccaccatcttctctgtgcgctccaggactcctcgctgacgggcgagctcctcggaagaggcgaccccaaccttctcggactcgtacatgagggccagggacctgctggtgctggcggccgtggcctcagccctgcggaggacctcctgccgcaagtactgctgcctgtccgcgggcgcgtcgggcccgtcggggaggtctcgggcgtccctccaaggggccggccgggcgccttcgtcctccccgtcgtcgtcgaacggattgtagcttttagggtaagctgacatggtgccggcgcggctctcggtctgggaaacagaaggaggagccccactgccgccgccgtccagggcctcgccccgcccgccgaccccgcggtcgtcgcgcgaac

SEQ ID NO: 14206 - RNA, 4419 nt, Homo sapiens
  source 1..4419: mol_type = other RNA
gctgggattacaggcatgagccaccgcgcccagccaggaaagaactttatacaagtctcatgctttatcttaaaaatatatgcaaatcaaaatatattcatgttcattttaatattaagggaatttccatttccaaagcatcaccgcccatcacagtagttccacggatcccagcttgagaactattaaatgaaaaaccaaaaaatgcaaatagcaggatagaaaagttgtaggtacattaaaatggttacacctaccaccaccactggggaatcctgtaagatgttaatggctgggaatgggggctcacgcctgcaatcccagaactttctggggccgaggcaggcagatctcttgaaccctgtctctacaaaaaatagaaaaattaggcggacatggtggccagtgcctacagtcccagctacaaagtgggctgagatgggaggattgcttgggcctgggaggacgaggctgcagtgagctgagatcgcaccactcctccgggcaagagtgaggctgtctcaaaaaaaaaaaaaaaaaaaaaaaaaaaaaaagggtgggttagcatagtggattttaggtaagtttactattttctttttggtaatgtagttttaccacttttattataaaaaatgtgtttagaagaatctggctgagttgctaagtctcccgtgtggtaacacaatttgaggcagatgaccacaatactagttttcaattttgatatttaaaaaaaaaaatttttttttgagatgcagtctcacgctgtcacccagactgaatgcaatggcatgatctcggcttactgcaaaccccgcctcccgggttcaagcgattctcctgcctcagcctcttgaatagctgggattacaggcacgcaccaccacagttggctaatttttgtatttttagtagacacagggtttcaccatgttggccaggctggtctcaaactcctgacctcaagtgatccatccgccttggcttcccaaagtgctgggattacaggcgtaagccaccgtgccctggccctcacctacattggttactttctctaagtcagactgggggtctgtctctgcagagtgctgggggagcgtgctccatgtgatgcacaggagccccccacattgcccccaaaggtgtgacttaaagttatctatcacaagggatgggaggttacttggccaacccagaaaccctaaataggtaaaatagctcattgagtgcctgtggccagcggggagcaacttcgtccctgcaccgcacaaaacttcacctcttcctactccgtccctgcaccgcacgaaacttcacctcttcctactccgtccctgcaccgcacgaaacttcacctcttcctactccgtccctgcaccgcacgaaacttcacctcttcctactccgtccctgtactgcacgaaacttcacctcttcctactccgtccctgtactgcacgaaacttcacctcttcctacttcgtccctgtactgcaagaaacttcacctcttccgaatctcaccaatgaaaatgtcctcaagtttatataaaatatctaacagaggcaaacaaaacaattcccttccttttctgatggtaaaatactgcaatacaatttgtttgcaatgcagtagttaaaattagtaacattcctgttccttttttttgattgagtttcactcctgttgcccaggctggagtacaatggcacgatcttgctcactgcaacctccgcctcccaggttcaaatgattctcctgcctcagcttcctgagtagctgggattacaggtacccactagcatgcctggctgatttttgtatttttagtagagatggggtttcactatgttggccaggccggtctcaactcctgacctcaggtgctccacccgcctcgccctcccaaagcgctgggattacaggaattatccactgcacctggccaaaactcctgtttctaatgatcaaaaaccagggctgtaggattagaagtcactattactggctgggtgcagtggctcacgcctataatgccagcattttgggaggctgaggcaggtagatcatgaggtcaggagtttaagaccagcctggccaagatggtgaaaccccatctctactaaaaatacaaaaaaaattagccaggcatggtggcgtgagcctgtagtaccagctactcaagaggctaagtaaggcaggagaatcacttgaacccaggaggcggaggttgcagtgagtttagattgtgccgctggactccagcctgggaaacagagactccatctcaaaaaaaataaaagaagtcactattacattattgatactcagctgataatcagtttaatgcgaaattgactaggctgagcacagtagaatcacaccgctctaaagcacttaaaattctctaattatatggatttgcccagtgattcataaccttagagtttaagaaaaattccttgcacatagtagatattccaaaatatatgttggataatcagtgttactgttgctaattcaccactcactgtaaaaagtgtgaaagtggccgggcgcagtggctcacgcctgtaatcccagcactttgggaggcggaggtgggcagaccatctgaggtcaggagttcgagaccagcctggccaacatggtgaaaccctgtctctactaaaaatacaaaagttagctggacctggtggtgagtacctgtaatcccacctacttgggaggctgaggtgggagaatcacttgaacccaggaggcggaagttgcagtgagccgagaatgtgccactgcactccagcctgggtgacagagtgagaccctgtctcaaaaaaaaaaaaaaaaaaaaaaaggtaaaagtgaaaccgattatgcacagcgggccttgtgactcttgagtggattttatttttgcactccaggatgcagtgaagacggtggaaggttcatcttcacaccgagggccctcagtgtcgaggtgactcccggcctgaggagggctgaggcatcctgaattttgagagttcgaggttgaggtctaagaaggtgtacgtgctgtagtcatgatgctgcaggttcttgtaggtagtgttgtcaaacggctcagcaggcactggggctggctcctgtgtgccgcctcggtcgtcccctggcgcggctgcatcttccatggcctcgccctcggcctcaagcttcagcgctgctgtcttttcatggaaaccgtggttattctcaacaggaactgtctccaaattgcttggtggtatctgatcttccacgattgcctgtccacccttcaggtggccttctattccctgcgtccctgaggtttcctttctgggcaggggaggggccgccttgcgctggggctctggcacgggtttttccagatgcccctctgccgccccaggaggactggcttgcagctgcccctctgctctggcctcttctgccaacacagcaggcgctgggctgcccttcggtggcgcagacaaccctgattttgtgtggacaggtaagggtcctttaacttcaaatggcttttggctttctttatctatttcatttaatctaaatgttttctgcaattgtttttcctttaaactttgcttcaaaaactcttcatctacttgagatctgggcattgtggtttttggtctcgcattttccctgccttctgatggcttagcaggggaccctttcttctttggctggtggggcttctctggatcagtaatgtccacatgcggcttctgcagcaaggttttctcttttgctgatactgtaactcggggggctctgttttcaaaggaatgagaggcctctggttttcgaagcccccctctgcctttgctcaccactcgaggagtgacctctgaaacgtcagcctcatcatcagattcagaatcagaggagctggaagaggatgaagacgaaggcgacgtcactttccgacccacctgacgagcttctgaatcagagccctgttttctgaatggagacagaactttctgtggaaactctaccaaagtctttcttgacaaaaatttcggaaccccttcatctgtgaatagcacgctgccactgggactgggactagctaccttcctgcccttattcacagctggcgggtaagaactgggtgaagataagtttttagacaattcagctgctgtctgggtggctaggagcttgcccctctcctttggttccactacattttttggtggactttgcttcttggaattctgtggctgacccttttcactcttccctgattccgcagacaaagaaaccgtagaagcaagtcctcgaaacacctgggcttcctggagcatagtcttcagcgccccggctcgtccttgccgcagcaaacacggggcagccatggcggtgacagcgggcgcaccaagc

SEQ ID NO: 14207 - RNA, 3324 nt, Homo sapiens
  source 1..3324: mol_type = other RNA
gctgggattacaggcatgagccaccgcgcccagccaggaaagaactttatacaagtctcatgctttatcttaaaaatatatgcaaatcaaaatatattcatgttcattttaatattaagggaatttccatttccaaagcatcaccgcccatcacagtagttccacggatcccagcttgagaactattaaatgaaaaaccaaaaaatgcaaatagcaggatagaaaagttgtaggtacattaaaatggttacacctaccaccaccactggggaatcctgtaagatgttaatggctgggaatgggggctcacgcctgcaatcccagaactttctggggccgaggcaggcagatctcttgaaccctgtctctacaaaaaatagaaaaattaggcggacatggtggccagtgcctacagtcccagctacaaagtgggctgagatgggaggattgcttgggcctgggaggacgaggctgcagtgagctgagatcgcaccactcctccgggcaagagtgaggctgtctcaaaaaaaaaaaaaaaaaaaaaaaaaaaaaaagggtgggttagcatagtggattttaggtaagtttactattttctttttggtaatgtagttttaccacttttattataaaaaatgtgtttagaagaatctggctgagttgctaagtctcccgtgtggtaacacaatttgaggcagatgaccacaatactagttttcaattttgatatttaaaaaaaaaaatttttttttgagatgcagtctcacgctgtcacccagactgaatgcaatggcatgatctcggcttactgcaaaccccgcctcccgggttcaagcgattctcctgcctcagcctcttgaatagctgggattacaggcacgcaccaccacagttggctaatttttgtatttttagtagacacagggtttcaccatgttggccaggctggtctcaaactcctgacctcaagtgatccatccgccttggcttcccaaagtgctgggattacaggcgtaagccaccgtgccctggccctcacctacattggttactttctctaagtcagactgggggtctgtctctgcagagtgctgggggagcgtgctccatgtgatgcacaggagccccccacattgcccccaaaggtgtgacttaaagttatctatcacaagggatgggaggttacttggccaacccagaaaccctaaataggtaaaatagctcattgagtgcctgtggccagcggggagcaacttcgtccctgcaccgcacaaaacttcacctcttcctactccgtccctgcaccgcacgaaacttcacctcttcctactccgtccctgcaccgcacgaaacttcacctcttcctactccgtccctgcaccgcacgaaacttcacctcttcctactccgtccctgtactgcacgaaacttcacctcttcctactccgtccctgtactgcacgaaacttcacctcttcctacttcgtccctgtactgcaagaaacttcacctcttccgaatctcaccaatgaaaatgtcctcaagtttatataaaatatctaacagaggcaaacaaaacaattcccttccttttctgatggtaaaatactgcaatacaatttgtttgcaatgcagtagttaaaattagtaacattcctgttccttttttttgattgagtttcactcctgttgcccaggctggagtacaatggcacgatcttgctcactgcaacctccgcctcccaggttcaaatgattctcctgcctcagcttcctgagtagctgggattacaggtacccactagcatgcctggctgatttttgtatttttagtagagatggggtttcactatgttggccaggccggtctcaactcctgacctcaggtgctccacccgcctcgccctcccaaagcgctgggattacaggaattatccactgcacctggccaaaactcctgtttctaatgatcaaaaaccagggctgtaggattagaagtcactattactggctgggtgcagtggctcacgcctataatgccagcattttgggaggctgaggcaggtagatcatgaggtcaggagtttaagaccagcctggccaagatggtgaaaccccatctctactaaaaatacaaaaaaaattagccaggcatggtggcgtgagcctgtagtaccagctactcaagaggctaagtaaggcaggagaatcacttgaacccaggaggcggaggttgcagtgagtttagattgtgccgctggactccagcctgggaaacagagactccatctcaaaaaaaataaaagaagtcactattacattattgatactcagctgataatcagtttaatgcgaaattgactaggctgagcacagtagaatcacaccgctctaaagcacttaaaattctctaattatatggatttgcccagtgattcataaccttagagtttaagaaaaattccttgcacatagtagatattccaaaatatatgttggataatcagtgttactgttgctaattcaccactcactgtaaaaagtgtgaaagtggccgggcgcagtggctcacgcctgtaatcccagcactttgggaggcggaggtgggcagaccatctgaggtcaggagttcgagaccagcctggccaacatggtgaaaccctgtctctactaaaaatacaaaagttagctggacctggtggtgagtacctgtaatcccacctacttgggaggctgaggtgggagaatcacttgaacccaggaggcggaagttgcagtgagccgagaatgtgccactgcactccagcctgggtgacagagtgagaccctgtctcaaaaaaaaaaaaaaaaaaaaaaaggtaaaagtgaaaccgattatgcacagcgggccttgtgactcttgagtggattttatttttgcactccaggatgcagtgaagacggtggaaggttcatcttcacaccgagggccctcagtgtcgaggtgactcccggcctgaggagggctgaggcatcctgaattttgagagttcgaggttgaggtctaagaaggtgtacgtgctgtagtcatgatgctgcaggttcttgtaggtagtgttgtcaaacggctcagcaggcactggggctggcttttttggtggactttgcttcttggaattctgtggctgacccttttcactcttccctgattccgcagacaaagaaaccgtagaagcaagtcctcgaaacacctgggcttcctggagcatagtcttcagcgccccggctcgtccttgccgcagcaaacacggggcagccatggcggtgacagcgggcgcaccaagc

SEQ ID NO: 14208 - RNA, 1989 nt, Homo sapiens
  source 1..1989: mol_type = other RNA
gctgggattacaggcatgagccaccgcgcccagccaggacatcttttttatggccgcctagtattccatggtgtatatgcaccacattttctttatccagactgctatcgacgggcatttaggttgattccatgtctttgctaaataccagacctatggctttttaacaaaaaaaaattttctatgttcttcagggctgaattacatgccttcagatatcagatctctacatggctttctcttcctatatttgaggtctctgttcaaatataagagaaatctttcatgacaaaaacttattctgtgacagcccctcctttcatctctttatttctttaccctgccctattgttcttaaaagtgtctctcgctatatattgggggtttgctatgccctcgtagcccattataatatcatctttgtgagatcaaggtctttgttcactgctgtatatttcacatctaggacccttggctggcacagagtagacccttcaacaatcatatgttgaatgaatggttcaggtgataaataatgaggccctgatccacatggtgtatctatcaactattcactgagtcattaaagtagtcattctgcaaatctttgggttccttccaaatgcttgtagcaacttagtaggtgttggggatggagcaggtaacgaaactccacattagacaagtgtaatgaatataagtaagtaaatacctagaaggatgttagagaggaataagggcttagagaaaagaagtaagcagagatgagggataggaagtgttggggtgcagttaggagaccgaaattatctacaggatggctagagagagactctgaggtggtgacatttgaataaagaagaaagagtttcttagtgtggctctcctaatagtctctctggccctagcctcctccccctcaagcctcctcccgtttgagagggtaatctgtttctaacatgaaaggaatctttttactctcctttccagaagtccttcagtgttctcctgctgacttgcagataattttgtgacttgaacgtcatcatggtttgaattctgccttcctgcccatctctttctgcctgttatttgtcttcacatcatgacatttgttctctgggagttttatagtgatttggattctctggctaatagagctcagtcaccctccagggctcagattaagctacgtttgtgtagaacccctgcattccactgtgggcttatgagcccattcctcatgccgctaaaggatgctgtgcactactctggcatttagccatgtatagtggaattgccagcttcctcatcactagactgtgagcatcttgaggctggggaattgcatctcttttagtaaggttcccacaagtcttcactgagttaataaactcatctatttaatgaagtagtaataaattcacctgtctagtgctaattatgcaggcagtaaaatagtgttcattctcagtattttaagggacacattctgtgggttctgtaacagtgactcatgtcgtcgctgactttgaagagcagagagtactttcctaagatggtatttaacaaaatccagagatgcttttccttccaaagatgactctgatcttgcccaaggacagcaaatatggtgaaagacctttataactcacagtcctggagactgggaagtccatgatcaagtcactggcaaatccaatgtctaatgaggccactcttactggttcgcagaagctgttgtcttgtatcttcctagaataccaaccgtggaccatacgctggagctcgccaacttctcctctcacacgcaggtttgaggctttgaggtctgcatgcccgtgctctgccttctccagccgagactcaagattccactcgcctcctctaaacacgcaggacgacctgaaatcatagcccttaatagagcaagtcaaccaacggtacagatggtcaagctcttgctcatgtgccctccgagcataggct

SEQ ID NO: 14209 - RNA, 2434 nt, Homo sapiens
  source 1..2434: mol_type = other RNA
gctgggattacaggcatgagccaccgcgcccagccagtggcatgttattaagagatgtggataccagtttctccaggagatcacagagctttccctgtaggagtaatcaatggaggcatccttgttggggaagggtcttggtggtagatgctggtctgaaaattgaccaaggccttaagtaaaagttaggagctgtatttccagagtagaaaaagagagagacagagagagagagagagggagattctaggcgtgaagaaagcccaagagctcacaaaatcttgagcttgggatagaaatcagactggaccaagtggagggttatagtggacagtgctcatttaacaaaatattttgtttataaatttattatttgatgttttaaaaacgtatcaagaaaacattatgggcaaaatcagaacacagttggacttccttacatttatgttattttttttccttttttcaattgatacacatatttgtacatatttatggagtacatgtgatattttgttacatgcatggaatgtggaatgatcaagtcaaggtatttagggtagacatcacctcaagtatttatcatttttatatgttgggaacatgtcaagttctctcttctagctattttgaactagacaatacgttgttactgactatagcaccccactgtggtatagaacattagaacttattcctcctatctaactgtatgtacccaccaactaagcactctcttaatccccttccccaccagcacaccttcgcagcatctggtatctatcattctcctctctacctccataagatcaactttttttagcttccatatatgagtgagaacttgcaatgtttgtctttctctgacagccttatttcacttaacataatgacctccagttccattcatgttgctacaaatgacaagattttattccttttttatggccaaatagtattctatttgtgtatttatatcacatttttaatccatttgtccattgatggacacttaggttgatcccctatctttgctattgtgaatagtgctgtcgtaaactgagagcacaggtatgctgtgatgtactgaactcctttcctttagaaaaataccccatagtgggattgctgggtcatatggtagttctatttttagttttttgagaaatctccgtactgttttccataatggctgtactaatttagattctcaccaacagatccttgccagcatctgttactattttttttttgtctttttaatagtagccattctaacaggggtaagaaaatgtctcattgtggatttcgatttgcatttccctgatgattagtgatgttgagcattttttcatgtacctgttggccatttgtatgtcttcttttgagaaatgtctattcatgtcctttgctcactttttaatgggattatatgggttttttttcaactgttgggttgtttgagttccttgtacattctggatattagtcctttgtcacattaatagtttgcaaatattttctccaattcaccaggctgtctcttcacactgttgattgtgtgtagatgctgtgcagaagctatttagttcaacatagtcccatttgtctagtgttgtttttgttgcctatgcttgtgatcctgttttatatttatggaggatagaggtgagacatcataatcatatcagtgttaaggaccttgaaaggttgaatgcagatctttagtagcacataaagctgggactatattttggaagacttgaattccaagtgaagcagttggaccttgcatatcttgatgtgcaaagggctttgaggacaatgactacctcaagttctctgggtctctggagaaaaatatttctgattttacatacctagtctaatattggatttcgtatcttttactgcatagtgtacattttaaaaactacatatgtaagagttttctggtggtagaaattatgcctctttgtttcattactcttgttcattggtattagttggaagagataatgtccctttaagtgcaaaccctcccttgaagaataaatcctaaaacaactggtgatgtttattgcttctattagcttgataatcttaagacaatcttgatgccatttacacaactttttcattcctccatgttaccgggacactacttagccattatgggttgttacattgtgcttaggatggtgaagatctgacaacatggtgtcctgagtcacacatatcctgatgatcgcatggctaactgggagctgtgctcaccgccactgcccagcatcaagagagggtaccacgccacatatcgctagcccatcagccatccatcccttcaccatccagaagaaacacttaacatttaattgtatattgttagctttccaggcttgtgtgtatgtgtgtgtgtaatttttcatttaaa

SEQ ID NO: 14210 - RNA, 2500 nt, Homo sapiens
  source 1..2500: mol_type = other RNA
gctgggattacaggcatgagccaccgcgcccagccagtggcatgttattaagagatgtggataccagtttctccaggagatcacagagctttccctgtaggagtaatcaatggaggcatccttgttggggaagggtcttggtggtagatgctggtctgaaaattgaccaaggccttaagtaaaagttaggagctgtatttccagagtagaaaaagagagagacagagagagagagagagggagattctaggcgtgaagaaagcccaagagctcacaaaatcttgagcttgggatagaaatcagactggaccaagtggagggttatagtggacagtgctcatttaacaaaatattttgtttataaatttattatttgatgttttaaaaacgtatcaagaaaacattatgggcaaaatcagaacacagttggacttccttacatttatgttattttttttccttttttcaattgatacacatatttgtacatatttatggagtacatgtgatattttgttacatgcatggaatgtggaatgatcaagtcaaggtatttagggtagacatcacctcaagtatttatcatttttatatgttgggaacatgtcaagttctctcttctagctattttgaactagacaatacgttgttactgactatagcaccccactgtggtatagaacattagaacttattcctcctatctaactgtatgtacccaccaactaagcactctcttaatccccttccccaccagcacaccttcgcagcatctggtatctatcattctcctctctacctccataagatcaactttttttagcttccatatatgagtgagaacttgcaatgtttgtctttctctgacagccttatttcacttaacataatgacctccagttccattcatgttgctacaaatgacaagattttattccttttttatggccaaatagtattctatttgtgtatttatatcacatttttaatccatttgtccattgatggacacttaggttgatcccctatctttgctattgtgaatagtgctgtcgtaaactgagagcacaggtatgctgtgatgtactgaactcctttcctttagaaaaataccccatagtgggattgctgggtcatatggtagttctatttttagttttttgagaaatctccgtactgttttccataatggctgtactaatttagattctcaccaacagatccttgccagcatctgttactattttttttttgtctttttaatagtagccattctaacaggggtaagaaaatgtctcattgtggatttcgatttgcatttccctgatgattagtgatgttgagcattttttcatgtacctgttggccatttgtatgtcttcttttgagaaatgtctattcatgtcctttgctcactttttaatgggattatatgggttttttttcaactgttgggttgtttgagttccttgtacattctggatattagtcctttgtcacattaatagtttgcaaatattttctccaattcaccaggctgtctcttcacactgttgattgtgtgtagatgctgtgcagaagctatttagttcaacatagtcccatttgtctagtgttgtttttgttgcctatgcttgtgatcctgttttatatttatggaggatagaggtgagacatcataatcatatcagtgttaaggaccttgaaaggttgaatgcagatctttagtagcacataaagctgggactatattttggaagacttgaattccaagtgaagcagttggaccttgcatatcttgatgtgcaaagggctttgaggacaatgactacctcaagttctctgggtctctggagaaaaatatttctgattttacatacctagtctaatattggatttcgtatcttttactgcatagtgtacattttaaaaactacatatgtaagagttttctggtggtagaaattatgcctctttgtttcattactcttgttcattggtattagttggaagagataatgtccctttaagtgcaaaccctcccttgaagaataaatcctaaaacaactggtgatgtttattgcttctattagcttgataatcttaagacaatcttgatgccatttacacaactttttcattcctccatgttaccgggacactacttagccattatgggttgttacattgtgcttaggatggtgaagatctgacaacatggtgtcctgagtcacacatatcctgatgatcgcatggctaactgggagctgtgctcaccgccactgcccagcatcaagagagggtaccacgccacatatcgctagccctcaccacctgctgaaagtgtccacatcatggaaccctctggaatgtggtcttcttttctccaagtgactcatccagcctccgcactgttaccagaaatacctttccaacacacaaatcagattaggcctctcccctgcttcaaacaatttcaaatctcttggcgccagctttc

SEQ ID NO: 14211 - RNA, 5658 nt, Homo sapiens
  source 1..5658: mol_type = other RNA
gctgggattacaggcatgagccaccgcgcccagcccagagaggcctcttttaaaaaatgttttaaaaatcaaaagcacaggccaagtcagaaagcctccttgtggtcttcctggccagcaggagatttttcttttcttgtctacccttgtgctgagagtgttggttattatagagcttgagcattatgtgcagagctcagttgtcacttcatgttatatgggctgaaggctttgagtggctattaatatctaaacttgttgattgagactgctaccctcctccccaccacccagcctcctgcaccagagtcatttcaagcttctggtttttattctattgggaatgagatttctttcatttccttgtttaggccctgaaggataagttttcctcttattttcttgtgcccttagccatatatttaatagggaagaaggtaagttcctctcttgtttcataattttctatgtagataacaactaaagggaacacagagcataaaagttttgaggttgtatttatttcaatatggaagtcttgttttccagatctgcagcgtccaagagaaccttctgaatgatgggaatgttttctactctgtccagtgtggcagacccttgccacatgtagctattgagcatttgaaatgtggctgatatgtctgataaactaattcttaaatattatttaattgtaattaatttaattaaaatggtcagatacaattagtggttattgtatttgacaacacagttctaagtggtaatattctttgtcccctaggtgggtttatgtactggtaaaccagtgttgtcttgaaaatctgatatttttgaggatgtaaatatatttgaggattaaatatttgagatgtgacttcagaatatatgtcaccacaggctgggcatggtggctcacacctgtaatctcagccctttgggaagctgaggcaggagggtcacctgaggccaggagttggagaccagcctgggcaacacagcaagactctgtctctctgtttaaaaaaaaaaattagcctgacatggcagtgtgcacctgttgtcctagctactcaggaggctgagtcaggaggatcacttgagctccaggagtttgaaggtgcagtgagctacgactgtgccactgcattccagcctgggtgacacaacaagatcctatctctaaacaaacaaacaaggaatgtatgccaccacaaaactgtatagcccattattttgataatcaggtatttcttgtctgatttgtctttctgggaattttcaaagatctacagtgatcaagtttaagtgcacattcttcccattgccagtttctgatctgaagtcagagaatcactttctgaaagctttttcaagagtatttatgaagtaataaagtgtgaagaaatcctgaggataaataacaagaagcataaatatacatatttagaatgcaacataatatgtttaagattacaatttggcggcagggcgcagtagctcatgcctgtaatcccagcactttgggaggccgaggcgggcggatcacgaggtcaggagatcgagatcatcctggctaacacggtgaaaccctgtctctaataaaaaaaaaaaaaaaaaaaaattagccaggcatggtggtgggcacctgtagtcccagctactcaggaggctgaggcgggagaatggcgtaagtaaacccaggaggcagagcttgcagtgagcctagatcacgccactgcactctagcctgggcgacagagcagcgagactctgtctcataaaaaaaaaaaagtacaatttggcctatctttgaactaaaaagtttactggtaccctgaaaatatgtataagtaaaaacatgaatgcttcatatgatttattaaaagcattttatgaaaaaaaaacaaaaacacaaaacctctccaggtatggtggctcacgcctgtaatcccagcactttgggaggctcaggtgggtgggtcacctgaggccagcagttcgagaccggcctggctaacatggtgaaaccttgtctctactaaaaatataaaaattagctgcgtgtggtggtgcacacctgtagtcccagctactcaggaggttgaggcaggagaattgcttgaactcaggaggcggaggttgcagtgagccaagatcgtgccactgcactccagcttaggtgacagagtgagactctgtctcaaaaaaaaaaaaaaaagacaaaacaacaacaaaaaaaacccaagcctactgatctaggcttagagtgggcttacactttcaaagggcattgtattatacaaaatatctctcaaaaaaaatttttttggccataggtagagattaagaaggctaaaacaaaaatgcatatatgaattttaatgataacacatatatgtatatttgaaaacaaggccacataagcctggctggcacattgggccattttactggctggccttcaaaaataaagattacaaaaaatttatccacatacacttttttatatccctaaagattacaaaaaatttatccacatatacttttttatatccctgtataaaattgatgccaacatgtttggcattttagaaagacactcaaacagattctggaaaaagaaatcgcttcatgggatgaacagactaggtcgcaaatgaaaaagctaaacatttgttttttaaaccacaccacaaatttccaggtaaaactgattgaaacttatgctcagagatattttcactgtacttacatgacttgaaaatctgtaagaaccaaagcccctaaattctactgaacatacttcaaacattttgcctagtaaaattttttttaacactctcaaaaaattttaaaaagaaacaaattttctctggaaaggattttcagcatcttgaatatatatattttctcagagtgtatgcagcccactcttctcttgataatcttcataaaaacgtctcaatgactcaggaattctaggtgtcacagtgctcaaggcctgagtgaaatgtcttttcatgatgagattggcttgaatgtcttcttccagagccagaagagctgcctctctgcagacagctacaatctctgctcctgagtatgcgtcggtttgaaggatgagttcatccaggtcaacttcattactgacaggcatggagtgaaactgcagcttaaatatttcccttcttgttgctgcatccggtaaaggcacatagatgattctatcaattcttccaggccgcatcaaagccttgtctatcctatctggacggttagtagctgccaaaatggtcacatcctttagctgttcaatcccatccatttctgttaagagctgagccaaaacacgatcggctacattcccagcacctaaagaactgcccctttcaactgctaaggcatccagttcatcaaagaaaataatggaaggcgccactgctcttgcttttcggaaggtctctctaactgctctttcagattcaccaacatatttattcattaattcaggcccctttatagctagaaaattcagtccactctcattggccaaagcctttgctatcattgttttagagcacccaggtggcccatagagaagaactcctttaggtggctgaatacccattcgaatgaaagactctggatgttttaagggccattccacagcctgttccaacttcagtttgatactttccagtcctcctatatctgaccaggatacatttgggacatcaattgctatttccctcatggcactgggtctgatatcattcattgcctgcaagaaatccttcagagtaatcttcaccagtccagccaccttgacatcagggaggttaggctgttttttcaggattctccgcaaggcacagagacctgcttcattacacaagactttcaagtctgctccaacgtatccatgagcactatttgccagctgcagcagctcagcctcagtgagcaaatggggtacccttcgaagcagtttctggagaatatctagccggtcctgagcattgggaactccaatctcaatctctttatcaaatcgcccaggtcttcggagagcagcatccaaggcatgagggcgatttgtggccccaagaaccaacacttgtccttcacttacttctgaaccaatgccatccatcagtgttaagagtgaagccacaactcttttttccacttcattctgggccccctctcttttcggacaaagtgcatccagctcatcaataaaaataattgatgggtgtcgtagagtggcttcagcaaatatctgacgtaactttgcttcagtctcaccatagaatttgcttataatttcaggaccattaattacagaaacataggctccaacttcattagcaacagccctggcgatcattgtttttccagtacctggaggaccataaagtaacactcctctaggggcaggaattccataactcttgaaaagctcaggctgtttgaggggcaattcaattatttctctaattgctttcagctggctacttaatcctcctatcatgtcataagttactttgaattggttgtcttgctcttttgaatttttatcaatctctgtaaaattgactcttgttgttgaagaaataaaataaaaagtatcagtattgcactttgctcctatgctgaactttagcagtctctcttcttcagtaagttgctcatttccttctctggcagattcaaaattacatttaagacctgtgacttcctctagcataagtccactgccatctccagggctctgtgtaacatccagcaaaacatcactggctttatttgtaattctgtcatcaattggtttataaggagtacttcttgatgttgggatctgggtatcctccagatctaactggcttagctgtaaggataactccaggctactggtttccatgctggactgttcaaaggccattctttgggcatcagtgtcagagtcactctgaggccctcccaatatcatgccatctgcccctttcactcgcaatacttgcagcttgtacggtcgtccatagaatgtacaatacagaaagttgcctggtaaaacaatcttgccatctagttttctcaggatacaaccagtcagttcttcttcattaatttccatatctttgtcactcagtgccacatccatttcctcagcctgtagcacagcacccacaagaggctggacctggatggcatcaccaggcctcacacccacatttttctgtgccatttcactcaggccgaccttgcctccaggaaatcctgccataggccaggctgtatacacctcttgctttccgttcaaactagtaagcaacactggtcgacctatacatatatttgcagacttcatagtgttgagtccaagatgaataagggaattctggaatgttttaggaattttgtcatccttttctaataagttggtcaccgtcagagtcccggaggttgccgcgaagtctgatccagcagaaggagcccgtgcctccgcacaagaggaagcagcagagggcaaggacgaaccattttccgcgctttggttcaaccgctttctattcttcttggaagacatggtcacaaggtaccctagccgaagcagtagaaaagccgactcaatgtgcgcgcttcaactgagag

SEQ ID NO: 14212 - RNA, 5661 nt, Homo sapiens
  source 1..5661: mol_type = other RNA
gctgggattacaggcatgagccaccgcgcccagcccagagaggcctcttttaaaaaatgttttaaaaatcaaaagcacaggccaagtcagaaagcctccttgtggtcttcctggccagcaggagatttttcttttcttgtctacccttgtgctgagagtgttggttattatagagcttgagcattatgtgcagagctcagttgtcacttcatgttatatgggctgaaggctttgagtggctattaatatctaaacttgttgattgagactgctaccctcctccccaccacccagcctcctgcaccagagtcatttcaagcttctggtttttattctattgggaatgagatttctttcatttccttgtttaggccctgaaggataagttttcctcttattttcttgtgcccttagccatatatttaatagggaagaaggtaagttcctctcttgtttcataattttctatgtagataacaactaaagggaacacagagcataaaagttttgaggttgtatttatttcaatatggaagtcttgttttccagatctgcagcgtccaagagaaccttctgaatgatgggaatgttttctactctgtccagtgtggcagacccttgccacatgtagctattgagcatttgaaatgtggctgatatgtctgataaactaattcttaaatattatttaattgtaattaatttaattaaaatggtcagatacaattagtggttattgtatttgacaacacagttctaagtggtaatattctttgtcccctaggtgggtttatgtactggtaaaccagtgttgtcttgaaaatctgatatttttgaggatgtaaatatatttgaggattaaatatttgagatgtgacttcagaatatatgtcaccacaggctgggcatggtggctcacacctgtaatctcagccctttgggaagctgaggcaggagggtcacctgaggccaggagttggagaccagcctgggcaacacagcaagactctgtctctctgtttaaaaaaaaaaattagcctgacatggcagtgtgcacctgttgtcctagctactcaggaggctgagtcaggaggatcacttgagctccaggagtttgaaggtgcagtgagctacgactgtgccactgcattccagcctgggtgacacaacaagatcctatctctaaacaaacaaacaaggaatgtatgccaccacaaaactgtatagcccattattttgataatcaggtatttcttgtctgatttgtctttctgggaattttcaaagatctacagtgatcaagtttaagtgcacattcttcccattgccagtttctgatctgaagtcagagaatcactttctgaaagctttttcaagagtatttatgaagtaataaagtgtgaagaaatcctgaggataaataacaagaagcataaatatacatatttagaatgcaacataatatgtttaagattacaatttggcggcagggcgcagtagctcatgcctgtaatcccagcactttgggaggccgaggcgggcggatcacgaggtcaggagatcgagatcatcctggctaacacggtgaaaccctgtctctaataaaaaaaaaaaaaaaaaaaaattagccaggcatggtggtgggcacctgtagtcccagctactcaggaggctgaggcgggagaatggcgtaagtaaacccaggaggcagagcttgcagtgagcctagatcacgccactgcactctagcctgggcgacagagcagcgagactctgtctcataaaaaaaaaaaagtacaatttggcctatctttgaactaaaaagtttactggtaccctgaaaatatgtataagtaaaaacatgaatgcttcatatgatttattaaaagcattttatgaaaaaaaaacaaaaacacaaaacctctccaggtatggtggctcacgcctgtaatcccagcactttgggaggctcaggtgggtgggtcacctgaggccagcagttcgagaccggcctggctaacatggtgaaaccttgtctctactaaaaatataaaaattagctgcgtgtggtggtgcacacctgtagtcccagctactcaggaggttgaggcaggagaattgcttgaactcaggaggcggaggttgcagtgagccaagatcgtgccactgcactccagcttaggtgacagagtgagactctgtctcaaaaaaaaaaaaaaaagacaaaacaacaacaaaaaaaacccaagcctactgatctaggcttagagtgggcttacactttcaaagggcattgtattatacaaaatatctctcaaaaaaaatttttttggccataggtagagattaagaaggctaaaacaaaaatgcatatatgaattttaatgataacacatatatgtatatttgaaaacaaggccacataagcctggctggcacattgggccattttactggctggccttcaaaaataaagattacaaaaaatttatccacatacacttttttatatccctaaagattacaaaaaatttatccacatatacttttttatatccctgtataaaattgatgccaacatgtttggcattttagaaagacactcaaacagattctggaaaaagaaatcgcttcatgggatgaacagactaggtcgcaaatgaaaaagctaaacatttgttttttaaaccacaccacaaatttccaggtaaaactgattgaaacttatgctcagagatattttcactgtacttacatgacttgaaaatctgtaagaaccaaagcccctaaattctactgaacatacttcaaacattttgcctagtaaaattttttttaacactctcaaaaaattttaaaaagaaacaaattttctctggaaaggattttcagcatcttgaatatatatattttctcagagtgtatgcagcccactcttctcttgataatcttcataaaaacgtctcaatgactcaggaattctaggtgtcacagtgctcaaggcctgagtgaaatgtcttttcatgatgagattggcttgaatgtcttcttccagagccagaagagctgcctctctgcagacagctacaatctctgctcctgagtatgcgtcggtttgaaggatgagttcatccaggtcaacttcattactgacaggcatggagtgaaactgcagcttaaatatttcccttcttgttgctgcatccggtaaaggcacatagatgattctatcaattcttccaggccgcatcaaagccttgtctatcctatctggacggttagtagctgccaaaatggtcacatcctttagctgttcaatcccatccatttctgttaagagctgagccaaaacacgatcggctacattcccagcacctaaagaactgcccctttcaactgctaaggcatccagttcatcaaagaaaataatggaaggcgccactgctcttgcttttcggaaggtctctctaactgctctttcagattcaccaacatatttattcattaattcaggcccctttatagctagaaaattcagtccactctcattggccaaagcctttgctatcattgttttagagcacccaggtggcccatagagaagaactcctttaggtggctgaatacccattcgaatgaaagactctggatgttttaagggccattccacagcctgttccaacttcagtttgatactttccagtcctcctatatctgaccaggatacatttgggacatcaattgctatttccctcatggcactgggtctgatatcattcattgcctgcaagaaatccttcagagtaatcttcaccagtccagccaccttgacatcagggaggttaggctgttttttcaggattctccgcaaggcacagagacctgcttcattacacaagactttcaagtctgctccaacgtatccatgagcactatttgccagctgcagcagctcagcctcagtgagcaaatggggtacccttcgaagcagtttctggagaatatctagccggtcctgagcattgggaactccaatctcaatctctttatcaaatcgcccaggtcttcggagagcagcatccaaggcatgagggcgatttgtggccccaagaaccaacacttgtccttcacttacttctgaaccaatgccatccatcagtgttaagagtgaagccacaactcttttttccacttcattctgggccccctctcttttcggacaaagtgcatccagctcatcaataaaaataattgatgggtgtcgtagagtggcttcagcaaatatctgacgtaactttgcttcagtctcaccatagaatttgcttataatttcaggaccattaattacagaaacataggctccaacttcattagcaacagccctggcgatcattgtttttccagtacctggaggaccataaagtaacactcctctaggggcaggaattccataactcttgaaaagctcaggctgtttgaggggcaattcaattatttctctaattgctttcagctggctacttaatcctcctatcatgtcataagttactttgaattggttgtcttgctcttttgaatttttatcaatctctgtaaaattgactcttgttgttgaagaaataaaataaaaagtatcagtattgcactttgctcctatgctgaactttagcagtctctcttcttcagtaagttgctcatttccttctctggcagattcaaaattacatttaagacctgtgacttcctctagcataagtccactgccatctccagggctctgtgtaacatccagcaaaacatcactggctttatttgtaattctgtcatcaattggtttataaggagtacttcttgatgttgggatctgggtatcctccagatctaactggcttagctgtaaggataactccaggctactggtttccatgctggactgttcaaaggccattctttgggcatcagtgtcagagtcactctgaggccctcccaatatcatgccatctgcccctttcactcgcaatacttgcagcttgtacggtcgtccatagaatgtacaatacagaaagttgcctggtaaaacaatcttgccatctagttttctcaggatacaaccagtcagttcttcttcattaatttccatatctttgtcactcagtgccacatccatttcctcagcctgtagcacagcacccacaagaggctggacctggatggcatcaccaggcctcacacccacatttttctgtgccatttcactcaggccgaccttgcctccaggaaatcctgccataggccaggctgtatacacctcttgctttccgttcaaactagtaagcaacactggtcgacctatacatatatttgcagacttcatagtgttgagtccaagatgaataagggaattctggaatgttttaggaattttgtcatctaccttttctaataagttggtcaccgtcagagtcccggaggttgccgcgaagtctgatccagcagaaggagcccgtgcctccgcacaagaggaagcagcagagggcaaggacgaaccattttccgcgctttggttcaaccgctttctattcttcttggaagacatggtcacaaggtaccctagccgaagcagtagaaaagccgactcaatgtgcgcgcttcaactgagag

SEQ ID NO: 14213 - RNA, 12922 nt, Homo sapiens
  source 1..12922: mol_type = other RNA
gctgggattacaggcatgagccaccgcgcccagcccatatacttaagctgacttttaagagattttgaatatatatgtaaaaatcaccatgactggctctatggcaaggtaggtgagactaatatttagagtttttttaaagtgctctcaaagttggatgttctatacctcatacatttttgaaaaatcttttggtcttcaaaatctgggtcttgtgaaatttggatgctcaaaacaaaacaagcctaggcaaaccaacaaactcagctatgataataaaagtttcctattactacaagatgcttgggtgtaaacaaatgatttcttgaaggaagagataaactactcaatgattcaaagtctctgaatcaggagtgaactgaagtgagatagggaaaagaggttttccttccatgaacagggaatccacctttattttaaagtatgacttgttttttgtttttgaacaaagaaaaaataatccttacaaagtattttaaatgggatagtttttttcgatgatacataaaagcacaatatagtagcagggataatggttacattaagtgcttaaagtaagtgcttcctccttaactccacccgatttgcatgccttaccactttcttttttttttttttttctttgagacagggtctcgctctgctgcccaggctggagtgctgcggcacggccttaccactttctgccatgcgctacttaggaatacgttctccagttaggctctgtagactcagagtaccttgcacactggtgctcattgtgcattttgtgtcatcagtccgctgaatgaacatagtaggaaatcatttttgggaggagtgggatctggggtgataaatcatattttcacttaaattatttaaagtcagtttctctgctggttacaagagtttaagctttggctaacttaataattagctcatgcactaaactggaagctttgattatcctaatgagtgtgaaagaatttcaaagaaaggggagctgtgggtctcgcactgtggtgctgccaagatgtggttaaactcagagcacctgactgtatagttccaagtcgtctttgcagtgcctctagccgagtgatataatctgttagggctctgtcaggatcgtaattctgaagctgagaacatgctaaagaaccaggattgaaatcagctggagtgcctgggtacctattctgaaatggtaaaggggacctaatatagtccagatctgatcttgagcgatacgtagtatgtcttggttctccatataactccagcccaccagaagaatgataaaatgagtcagtcttttctgcaccttgattcagtccaaagccatctctgttaatattgatggaaacagaacctgtgactcgatgccaccgtcgaaccaaaaatttcattctggaaattgcaatggatactctgacggccgaccgaaacctggtgaagccctttgggcgattggtgatcacctctagatccgtgaaagctggctgcccccccatccgggcaagcagggccaaggtggcatcttcacattcctggaacccacccagtaacagcagcaggtatttcttctggtaaatgagagcctttcgaaaactttctgccctcaagtatttaccataaattctctttaaagtgacatgttcagaatcagggctcagagtttgaagtaaagagtcatttcttagttcagctttcagtttgtatacttcagcctctgcccttttcaaagatttctggagagtcaatttttctctgttccatacttctttttcagaggcaatgatggcttcaatgttggcaccaccattcaatgaaaacctggaagaattatctctaccagctcctgtctgtcgataccacctgatctgctcttccagcttcataaccatgttccttaagtcattcttctcttcagtcagttgactgatatgccctgtcagctcagcattttgtctcagtagtctttcagtcaatgagccacaagaagtacttggggacaccaagctgggctcttcaccttgctggccagttaatttctgtagttgtaaaataatttcatcaatattttcctgaacccaaatgaaatcttcatcatctgctgtttcaaactgtagtctctcagaggctttctggggtagaacctgtagttttgaagctacacattgaagcttttgtctgatcatttctaattcatgattacagccggttcctcctccattcatttcaatcaatttagcgtagtttgattcttttgtttctccttctattttctgttgaagaacccaatttctagttctatcactggttaagctccacgtggttggctcattaaggttctgatacagaattcttctactttctcgtttttcttctcgttctagttcttgcttctggaattcctgcatgattccttgtagtcgctgtccttcaaggtctaacttataaacttgttgtcttttctcttccagctggcgctgaagatcttccactttggactggagctcatgcatttttttctgtccctcagtgttggcctcctgttctgtctgcagtgttttcctgtgaacctgcctatctttttccatttgctgtcgtgtttgcaaagaatccagtttatatttttcagtctcatttaacaattctactatgcgactgtgtttttcctctagctgtttctgcagctctttcagtaggtcctctgagggcaagggtggccgagactgtccagtaccatcactgctctgcagctgtgcgtgcaattcccgctccctatctagggtactactcatttcccgaattcgaactttctcagattcaagaagtacctgaagctctaagtttcgaccttgttcttctgacaactgggcatcatatagcattctctgtgattctattttttgctgggattcgttcagtagttgtttctgttgttccaaaagtagatttagctgaagattcctttgtttctgactctcaagtgaaaacttcagatcctcaagttcttctttatcccgttcttcactgcgtcccaacttggctttctctttctccaaagcccactggagctctcttgattttttctgttcacttgctaatgtgtcattaagcaaatgtacttcatctgtcttatctttaacttccaacctgaaagcctccaattcttttaggtgtttatgctgtgccttgagtgttgtttctagttccaatttagtttgtgcaagctcactcttcagttcagcaaccaccattttctcagaactcagctgctcctgcagttccgttgctctgtctttcatactgctgagctccacttgcatctccagcatttgagactgcttctgctgtatattatattccaagagttcttggcttggtttctcactctcttgttctcttttcagagtaattttcctaccattcatttgtgcatgcagtgcctgaatttcagataacaaactccttctatctgctttctggaggcattccatagctgcttgatattcaacaccctcggcttctctttgcagttgcatctttgtaattaaatcctttagagatgagattgtattgatgtaagcttttctctcttctagccaaggttctgaaacctgctgaatagaatggtcctctccatcactatagggagactcagtgagagaaagcacctgcatgccttcattatggacagctctcagtaatccctttattttctttggaaaggaatctgttgcactttcactttcttctcctcggccttctgatgctatgtcaaatccctgactgtgtgtaagataaattccctgaccccagtctgatccagaatcactggagcatatttctctagtctggtaagcatcagaatgtgctagctcaggaattgaggatccctctttacttctcagacactgtatcactgccttcaaggtaccacattcctctttcagtaactgaacggcaacatagtgttccctctttaaggtttcagtttctgaaatatgtctggattccatgtccaaaatttcagcagcatgtagttcttgcatcttctcaattttttcagtaaactgactgattatttcagtaacttcttctgaggaacattcactctgtaaattaatttgtattcctgcatttttaacaagaatttgtggagtctgattgctgctactgatcttcagagtcccatctgtctgggatgcaatgctcttactcagttttataggaagtggctcaaacatgcaggcctttttgctttcttgtacctcagtctcatcttctttttctaaaatggacaatttctcttttgcctctgcgaggtgatccctaacttggcttaagtctttctgaagagatgtcatatttgtttcttttaccaaaagctcttcttgaagtttttcagccttttctttataactggcaagttctgctttggtagccactgattcagctctaagagcctcgagttcattaaaaaatccactttcttcattgctatgaaatagctcagtagttgtcttgagaacttcaacatcttgagggcttcttttcttttctttctctctctgttttttctcattgccctccaatagcttctgtagttctagcagcttcttttctttttctaaaacatttttttctgcaatttctacttgttctttttctaaaatcaaactagtatgcatttcaacaacctggctttctaattctgatattctcaaggttaatgctgatatatctgaccccaactcatcttctcttagttgatttaaattctgaatatttgttctttcaggttctgatgaaattgtttgattatcttgacagaattttgcatattcctgaactgcctcaagttggatttgactgacaagagcagcagccactttttcttcaactattttctgtaggtttacaatcttcttttgaagcatttctgtttcaaactggccttgttcttgcatgtcttttatttgtttataacactgggtaagttctaagtcctttgcactaacagtgctctcaagttgtagcaaccttgtttccaaattaattatggaacctttgccattttcttcaaaagatttgaagtatgtctgattttctagggatttaagagcatcctctgtaaggactacttctagttcaggtttgtctttgctcagatgatctatagccacgttaacactattctctggtatgctttgaatcttttccacactttcacgttctctctttaagctgaataattcctgtgttagctgattcattttaaaattggtttctttaagtacatttttcatgaaggtcatttcttcattagcggtttctacttgctgttccaaggccagcttttcagctataaccacatccaattgatgttttaaactgtctgcttcttctgagagggaatgagcattcattgatgtcttctgtccaatatttgccaattcctgttgaagtttttcaatcacttcattgagctgctctatttcttcttctctatttctcttcacacattcttgatcactcatcaaacattctatttgggtttcaagatcccttatcagttcatttttttcttcaataaccttgttatctgttgtaattttaagttgctgctggagtttcgtaacttgttcatttaattggtcaatttctacctctttttcctgtattatttgagcaaatttcccaaatagcacatgttggtcttgagtagacatggcatcagattcctttatggcaagtcccagtttctccatgtcatccttaaataatttgttttcctgttcaagttcttgtaggcgggtagtagattcctttttctgtatttctaattgcatatgtaattgttgaacttcttcattcttattttccagttcttctctaaactgttctaattgctcttctaagtttgtaatctctttttcctttctgtctatggcatctcgttcagcctgcaattgtacttctagggacaattctggtttagcttctacagctccaaagtgttttcggtcctctaccttttgaaaagtatctgcactcacaagaagcgcctgctccagttctcttactctgaactccagtttctctatttcttcattcctttcttgtatatccctttgaagctgctctttagagagcaaaagctcactgcatttgtctgttttttctttcagatgatttgctaactgttcaacctctctagtttgatgttcactgataggctggaatcgaggaacaaccttaagttgctgttctagtttctgtatttcctgttggaatacatctctctcatgttctctgtcaatggcttgctcatctaaaaattttctcattttttctaactgcttttccaatgcttggttttgctgtcttaaatccattagttcagtatttttttcttgttccagctctataaacctactgacttgttcttccacatctatttctagagctttcacttgtttttgaaggtcatcacgtactttttcagcttgacattgtacttctagtttttccttcattaatttttctgtctcctgtagtaattctgctcctggtgctgcatcgactgcagcatctactagtcgttgttcaactgggcctgcctctgctttcatagcttccttttgtctggacagtaattctctttcttcttggatctgctgttgctctgcctccaattcttgcaacctgttacttgcacataacaactcctgctcaagacgatctattatatcagttttttcctgaatttgcctttcaaaaagagttttttcatctgcatagccatcaatgacgccctcagccttactgagctccacagctagctgttctctggccctggactcctcatgaaggcgctctcgaagttcctcttggcacttaagggactctgttgcttcttgtttctgtctaaatgactcacgcatcaactctgtctgtgtcactttcgcatgttcaagctgactgctagtttcacttatggcttctaggagtttttcaactgctgcttgtagtcgagagctaatgttcagcataagttcttcattttcagggtctatttcagttccagcaaaaccactcctcacaagtcgttgtgacagctctgttccttcctcagttacttttgaccacatgttaatgtcatttcttggcatatcacttccagaataagagggaatggattcatctgtaactcttgtatgttcctcatggacacatgactttacagatgcctctgcttctgacctccaaattaggctggcagatgactggcttttactagatctatctagaatcccaaggacatggcgaccaattgtttcttcaacagctgctgttgtctttacaacttctaagaggatcttcaaaagtctattattagctttctggagtgcatacactgtctttcttgtttgagttccatactgactgcgttccatactgatgatccaatggggaagccaaaatcttaggggccaaattcctccatgcaagctttcattagacaaaatctcaggaggcacatcttcaggttttctgtctaattccttttctttaaatgtttgttcttcaacttctccttggttttcatttccattctgtgtttgcgtactgctgttgcgcagctcacaacacagcttctctcttccagctaaagacagctgctttagtgcttccagctcctctaaaagcaccctctctctctctgaaaccaggttttcattatctatggaggatctctgggctaattgtctattaagtctcttaatctcttcttgtagctgttcctggtcttctcgctgtctctccatttgccgcatatgtgcttgccttaacaattccgttgcctgttgatgttcttggtattgtcgtacaagttcctgtctcatatcttccaactgttcttcattcaacattagttgtctagaagcatccatgcttgacactgaaatctcatcatgaatagactgtctaactataaatgttttatctttggagaacatttcttctgaaatagtcagcacacagtcctttgattctggtatatcatggggatcactatttgataataaaatttcctttccatgttctcctaactctttactaagtggtttaaattcttctttaaatttcacatccactgtctcaaaagtctgaaaaccaatttgatcctgtgataatttcatttcattaaaataatgttgttcttgctgacacacagcatgtgcttgctttgatgatgcagtattttcttttcccccagatattctagacagttcagtttgttgagcaaatgctatactcattgacacaataaccttagctacttcttcttctaattgttcttggtattgtttttcaagcaacttaacgatatttgtttcctctttcactccaaattcaccagaaaactctattgtaccatcaatattctttttcacacaacttccagggtacattgttctctgtgcatcagattctgtaattaccaccgaatcaacaggtaagcttggcggaaccgtggactcactaacagcttgaagcctcttctgtaaacagtggatctctgcctcatagttttgttcagtttctttcaactgttgctgcaaagaggatatgaggctttctaattcttgaacttgttcttcaagtttagttttttcaagatcttgcagagaagataacttgcttttatgattgacatcaatgtcttccaaattggtcatctgagaatggattgataaaaactctgtttcctcttttggaaggttttcttctccaaattcaagtttcataccatctgtctgctgtccccagatcttgcttagtcgtgtttgaagtaccaagagtttgttgtattcttctgttactttgttgagaagagtgtgcatattttcttgaaagtcttgaacttcatatctataatcttgtaattctggatcttcattttcagaaatgtaatcaccagaattctctttgtcttctgcatttacttcacattttaaagcaggagtataatattcaccaaggacactgcataaagtctgtaaaaaataagaacattcttcagacactgccttttgaagttttccaatgagcagatgtaaaggctttccttcatcacctgtttcttgtgttttcatagtctgtagttctaactggtgtattttctgaagttccttgatcttttcctcttgagcaaaaataagctcttctttaagactgcaaagagctttatctttttcattttccatatattcacgaacctgatccacatgagttgaataaaccagagagaggcaaatgcgttgggcttccatctgtagccttaaatcattctgttctgatttaagtacattgagttctttctgaagtttatcattttcacttggttgagttgctctaagtgatgattcctttgttacagatggtaagtgatccaaaatcaactgttcttgcttactttcttctccaacagtcatattttcaaaagaaactttatcttccaccattatttttgattcttcaccaaaacttttatttactttagaaactgatccttcagcacccctgcttgtcatggtcacaactccatctaataaagagcttacttgagtatcacatgactgtacattttctgccctgttgtggttaataatgatttctagctctctacatctcaatgaaacttgttctttctcttgctttaaagatttaacttcttcatttagaaaactaatctcaccatgtttctgtttcaattgttcagaaagatcagacagtctctgtgacagctctaatttctctcgcttggttacctcaagtttttccatgagttctgttgtatccttttcaacaacctcacccatttccaatgtttctgctacaaaagttttgtcttcatcaaagacagaacttttcattttcactgtagttggatttattctttgcaaatgaagctcttcattaagtgctttaagtttacttttatactctaattcctgtttatttttactgtcttctaaatcatcttttactttgagaaggcaagcatactcctcttgtaactcttgatagttaacttcaaagtttttttcagcaaatgaaaaagtgttcctttgcttttcaatctcttcatttagctgaatacattgttgtttgaggtcctcattttcctctataagtatttctatttctttttcccacacagagtctttggatttggacttaatggagtctaagaaaatcaatctttcttcttggctaacaggagtatgtattttcaacatgtcttcaagggttttcttttcatctttaagaatgctattctctgcttcaagttgtgcaaatttttcttgaagatcattctctttttccttcatctgtttttctaacaattctgttttaagttgtaattcttgaacttcttgttcaagtgtacccttttctttttcttcttgtctgagtatttcaatttctttttgaagttcattgatttgaagagtcatttcttctgactttgaatttacaagagactgctgtaaatcttttagctttgaaatttccaaaattaattgattctgcttagttatcaaattgtccttttcaaactgcatggtttctatcttttgactcatttcattctgtaaaccatctatctgctgtttatagtgaatgcctaaattatctttaagtttttcaatatttattcgatgttcaatttctaaatcttccttcagtttggaaagctcttcttcgtgactaaatagaagctgtgttctcagcctctctaattcagcttcttgtgattcagccattctgtctaacacagcattcttttctttttctaacatttcaagttttatcttgtaatttgtaacttctgcttcatgttttaattctagttcctttctggattcagatgcagaaacaatctcagctttcaaatcttccactgtactaagggacttatgtgcttcattaagtttactttcttgttcagctattgtctgtctagctctctgaatctgttcccttgaaaagctcaattcttcaacaaggtcttcaagctgtctctgtagagcacacttttcttctaaaattagtcctagttcttccttgagtttttccttttgagagttagtatcttgcaattttatattcagttcatttattgccacattcattaactttatctgatcttcattaactgtaatatttgaatatgaccttaaagcattctccatttctcccttatgccgtgttttcatttcctccatctgtgccatgtgttgtcttattaattcttgtttcatttgcactatctgctgcccatacatctcatccagctctgcccggagttgttctaactttctttgtgtttcttgttccattcgttgtactatatcagtttcgaactggctgtctttatgatttctcttctgaagttcttcgactgtccccattaactgttttatttcttcagaagactgtctttctttttgcttagaattagtcagctctaatttcatgttttttatttcttggttcttttgcacaatctgttcttgtaattctcctagtaatttatcagcagttgttaatttatcctttagctcaagagttttcttttcttcttctattatttttgtgtttaattcttcaatgattgtctccttttcctgtatttcttctttatttgagttttctacttttttatcttgttccatttcatatactttaattttctcttgcaagaaactaatttgcattgtgaagtcttctttctttttctgataatcttctaataagtggtcttgttcttcaagctgctgttgatgagtgaggatctgttgtttggcttgtagtaagtctgcagctgtgctactatgagtgctgtttctcagagtttcactagcctgtaattgctgaaattgaatctgtaatttttgactctgttctgtcaactctaaaaattctctcattgtctcatccttttctcttcttgcttgttgtaaattagcagtgagctgggttataatgccatctctttgtttaatggcagcttcaaattcttgtaactgctgcagtccttcagtcccataggtaaccctcatttcttccagctctctgtttagctcttcaatctcatgctgcttcccagccaactcactttccatcatctctagatgagtcggactgtcttgtgctccttgttcagaataagaatcatcaacaccaaattcttcttcccttaataaatttgtaggctttcctgttctcatcacaaaactgcaaccatttacctctgaactgcagtcatctgctgtggttgaaatttcactttccagttccacagagaagccctgctcatgactggttatttctccactatgtagagttctcattattgtagattcaggaatcacagttgattctactctctgagaactatttatgtacatttcattacactgtgattgatcaatattcaaatcatggtgtgctgacacatcatgtttactgcttgacgtttttctcttttttttctgcttcttggaaggactctgcccatccgactgagcttttctttgtcgaaactgggcaagcttggctttgccggcctccagcttcttctgtctctcctcgtcctccatggcctctgcaaggaaggcaggggaaaacaggggttgaggggtggttggggatagaaaggaaaggtcgatttggacggaggtgggacggcaagctccacggcctagagagccgattcggtccggcgctcccccgcccgaagtggaagcagtctccgcgctcactggcggatcgtcctcagccgcacgggaagcgccgtcaccgccgccgccgccgccatcttcgtctccacgta

SEQ ID NO: 14214 - RNA, 12970 nt, Homo sapiens
  source 1..12970: mol_type = other RNA
gctgggattacaggcatgagccaccgcgcccagcccatatacttaagctgacttttaagagattttgaatatatatgtaaaaatcaccatgactggctctatggcaaggtaggtgagactaatatttagagtttttttaaagtgctctcaaagttggatgttctatacctcatacatttttgaaaaatcttttggtcttcaaaatctgggtcttgtgaaatttggatgctcaaaacaaaacaagcctaggcaaaccaacaaactcagctatgataataaaagtttcctattactacaagatgcttgggtgtaaacaaatgatttcttgaaggaagagataaactactcaatgattcaaagtctctgaatcaggagtgaactgaagtgagatagggaaaagaggttttccttccatgaacagggaatccacctttattttaaagtatgacttgttttttgtttttgaacaaagaaaaaataatccttacaaagtattttaaatgggatagtttttttcgatgatacataaaagcacaatatagtagcagggataatggttacattaagtgcttaaagtaagtgcttcctccttaactccacccgatttgcatgccttaccactttcttttttttttttttttctttgagacagggtctcgctctgctgcccaggctggagtgctgcggcacggccttaccactttctgccatgcgctacttaggaatacgttctccagttaggctctgtagactcagagtaccttgcacactggtgctcattgtgcattttgtgtcatcagtccgctgaatgaacatagtaggaaatcatttttgggaggagtgggatctggggtgataaatcatattttcacttaaattatttaaagtcagtttctctgctggttacaagagtttaagctttggctaacttaataattagctcatgcactaaactggaagctttgattatcctaatgagtgtgaaagaatttcaaagaaaggggagctgtgggtctcgcactgtggtgctgccaagatgtggttaaactcagagcacctgactgtatagttccaagtcgtctttgcagtgcctctagccgagtgatataatctgttagggctctgtcaggatcgtaattctgaagctgagaacatgctaaagaaccaggattgaaatcagctggagtgcctgggtacctattctgaaatggtaaaggggacctaatatagtccagatctgatcttgagcgatacgtagtatgtcttggttctccatataactccagcccaccagaagaatgataaaatgagtcagtcttttctgcaccttgattcagtccaaagccatctctgttaatattgatggaaacagaacctgtgactcgatgccaccgtcgaaccaaaaatttcattctggaaattgcaatggatactctgacggccgaccgaaacctggtgaagccctttgggcgattggtgatcacctctagatccgtgaaagctggctgcccccccatccgggcaagcagggccaaggtggcatcttcacattcctggaacccacccagtaacagcagcaggtatttcttctggtaaatgagagcctttcgaaaactttctgccctcaagtatttaccataaattctctttaaagtgacatgttcagaatcagggctcagagtttgaagtaaagagtcatttcttagttcagctttcagtttgtatacttcagcctctgcccttttcaaagatttctggagagtcaatttttctctgttccatacttctttttcagaggcaatgatggcttcaatgttggcaccaccattcaatgaaaacctggaagaattatctctaccagctcctgtctgtcgataccacctgatctgctcttccagcttcataaccatgttccttaagtcattcttctcttcagtcagttgactgatatgccctgtcagctcagcattttgtctcagtagtctttcagtcaatgagccacaagaagtacttggggacaccaagctgggctcttcaccttgctggccagttaatttctgtagttgtaaaataatttcatcaatattttcctgaacccaaatgaaatcttcatcatctgctgtttcaaactgtagtctctcagaggctttctggggtagaacctgtagttttgaagctacacattgaagcttttgtctgatcatttctaattcatgattacagccggttcctcctccattcatttcaatcaatttagcgtagtttgattcttttgtttctccttctattttctgttgaagaacccaatttctagttctatcactggttaagctccacgtggttggctcattaaggttctgatacagaattcttctactttctcgtttttcttctcgttctagttcttgcttctggaattcctgcatgattccttgtagtcgctgtccttcaaggtctaacttataaacttgttgtcttttctcttccagctggcgctgaagatcttccactttggactggagctcatgcatttttttctgtccctcagtgttggcctcctgttctgtctgcagtgttttcctgtgaacctgcctatctttttccatttgctgtcgtgtttgcaaagaatccagtttatatttttcagtctcatttaacaattctactatgcgactgtgtttttcctctagctgtttctgcagctctttcagtaggtcctctgagggcaagggtggccgagactgtccagtaccatcactgctctgcagctgtgcgtgcaattcccgctccctatctagggtactactcatttcccgaattcgaactttctcagattcaagaagtacctgaagctctaagtttcgaccttgttcttctgacaactgggcatcatatagcattctctgtgattctattttttgctgggattcgttcagtagttgtttctgttgttccaaaagtagatttagctgaagattcctttgtttctgactctcaagtgaaaacttcagatcctcaagttcttctttatcccgttcttcactgcgtcccaacttggctttctctttctccaaagcccactggagctctcttgattttttctgttcacttgctaatgtgtcattaagcaaatgtacttcatctgtcttatctttaacttccaacctgaaagcctccaattcttttaggtgtttatgctgtgccttgagtgttgtttctagttccaatttagtttgtgcaagctcactcttcagttcagcaaccaccattttctcagaactcagctgctcctgcagttccgttgctctgtctttcatactgctgagctccacttgcatctccagcatttgagactgcttctgctgtatattatattccaagagttcttggcttggtttctcactctcttgttctcttttcagagtaattttcctaccattcatttgtgcatgcagtgcctgaatttcagataacaaactccttctatctgctttctggaggcattccatagctgcttgatattcaacaccctgttcttgtattctctgttccaaacagtttagtaaaccaactgcatctgtagtacctagagctgtcagctccgtccgaaatgctgctagtaaaacactacgctcttctaagaaaacttgttgaagggcaagcagtagttcacctcgccagtctgagaagctctcatgagattgagaactatcataaacctcggcttctctttgcagttgcatctttgtaattaaatcctttagagatgagattgtattgatgtaagcttttctctcttctagccaaggttctgaaacctgctgaatagaatggtcctctccatcactatagggagactcagtgagagaaagcacctgcatgccttcattatggacagctctcagtaatccctttattttctttggaaaggaatctgttgcactttcactttcttctcctcggccttctgatgctatgtcaaatccctgactgtgtgtaagataaattccctgaccccagtctgatccagaatcactggagcatatttctctagtctggtaagcatcagaatgtgctagctcaggaattgaggatccctctttacttctcagacactgtatcactgccttcaaggtaccacattcctctttcagtaactgaacggcaacatagtgttccctctttaaggtttcagtttctgaaatatgtctggattccatgtccaaaatttcagcagcatgtagttcttgcatcttctcaattttttcagtaaactgactgattatttcagtaacttcttctgaggaacattcactctgtaaattaatttgtattcctgcatttttaacaagaatttgtggagtctgattgctgctactgatcttcagagtcccatctgtctgggatgcaatgctcttactcagttttataggaagtggctcaaacatgcaggcctttttgctttcttgtacctcagtctcatcttctttttctaaaatggacaatttctcttttgcctctgcgaggtgatccctaacttggcttaagtctttctgaagagatgtcatatttgtttcttttaccaaaagctcttcttgaagtttttcagccttttctttataactggcaagttctgctttggtagccactgattcagctctaagagcctcgagttcattaaaaaatccactttcttcattgctatgaaatagctcagtagttgtcttgagaacttcaacatcttgagggcttcttttcttttctttctctctctgttttttctcattgccctccaatagcttctgtagttctagcagcttcttttctttttctaaaacatttttttctgcaatttctacttgttctttttctaaaatcaaactagtatgcatttcaacaacctggctttctaattctgatattctcaaggttaatgctgatatatctgaccccaactcatcttctcttagttgatttaaattctgaatatttgttctttcaggttctgatgaaattgtttgattatcttgacagaattttgcatattcctgaactgcctcaagttggatttgactgacaagagcagcagccactttttcttcaactattttctgtaggtttacaatcttcttttgaagcatttctgtttcaaactggccttgttcttgcatgtcttttatttgtttataacactgggtaagttctaagtcctttgcactaacagtgctctcaagttgtagcaaccttgtttccaaattaattatggaacctttgccattttcttcaaaagatttgaagtatgtctgattttctagggatttaagagcatcctctgtaaggactacttctagttcaggtttgtctttgctcagatgatctatagccacgttaacactattctctggtatgctttgaatcttttccacactttcacgttctctctttaagctgaataattcctgtgttagctgattcattttaaaattggtttctttaagtacatttttcatgaaggtcatttcttcattagcggtttctacttgctgttccaaggccagcttttcagctataaccacatccaattgatgttttaaactgtctgcttcttctgagagggaatgagcattcattgatgtcttctgtccaatatttgccaattcctgttgaagtttttcaatcacttcattgagctgctctatttcttcttctctatttctcttcacacattcttgatcactcatcaaacattctatttgggtttcaagatcccttatcagttcatttttttcttcaataaccttgttatctgttgtaattttaagttgctgctggagtttcgtaacttgttcatttaattggtcaatttctacctctttttcctgtattatttgagcaaatttcccaaatagcacatgttggtcttgagtagacatggcatcagattcctttatggcaagtcccagtttctccatgtcatccttaaataatttgttttcctgttcaagttcttgtaggcgggtagtagattcctttttctgtatttctaattgcatatgtaattgttgaacttcttcattcttattttccagttcttctctaaactgttctaattgctcttctaagtttgtaatctctttttcctttctgtctatggcatctcgttcagcctgcaattgtacttctagggacaattctggtttagcttctacagctccaaagtgttttcggtcctctaccttttgaaaagtatctgcactcacaagaagcgcctgctccagttctcttactctgaactccagtttctctatttcttcattcctttcttgtatatccctttgaagctgctctttagagagcaaaagctcactgcatttgtctgttttttctttcagatgatttgctaactgttcaacctctctagtttgatgttcactgataggctggaatcgaggaacaaccttaagttgctgttctagtttctgtatttcctgttggaatacatctctctcatgttctctgtcaatggcttgctcatctaaaaattttctcattttttctaactgcttttccaatgcttggttttgctgtcttaaatccattagttcagtatttttttcttgttccagctctataaacctactgacttgttcttccacatctatttctagagctttcacttgtttttgaaggtcatcacgtactttttcagcttgacattgtacttctagtttttccttcattaatttttctgtctcctgtagtaattctgctcctggtgctgcatcgactgcagcatctactagtcgttgttcaactgggcctgcctctgctttcatagcttccttttgtctggacagtaattctctttcttcttggatctgctgttgctctgcctccaattcttgcaacctgttacttgcacataacaactcctgctcaagacgatctattatatcagttttttcctgaatttgcctttcaaaaagagttttttcatctgcatagccatcaatgacgccctcagccttactgagctccacagctagctgttctctggccctggactcctcatgaaggcgctctcgaagttcctcttggcacttaagggactctgttgcttcttgtttctgtctaaatgactcacgcatcaactctgtctgtgtcactttcgcatgttcaagctgactgctagtttcacttatggcttctaggagtttttcaactgctgcttgtagtcgagagctaatgttcagcataagttcttcattttcagggtctatttcagttccagcaaaaccactcctcacaagtcgttgtgacagctctgttccttcctcagttacttttgaccacatgttaatgtcatttcttggcatatcacttccagaataagagggaatggattcatctgtaactcttgtatgttcctcatggacacatgactttacagatgcctctgcttctgacctccaaattaggctggcagatgactggcttttactagatctatctagaatcccaaggacatggcgaccaattgtttcttcaacagctgctgttgtctttacaacttctaagaggatcttcaaaagtctattattagctttctggagtgcatacactgtctttcttgtttgagttccatactgactgcgttccatactgatgatccaatggggaagccaaaatcttaggggccaaattcctccatgcaagctttcattagacaaaatctcaggaggcacatcttcaggttttctgtctaattccttttctttaaatgtttgttcttcaacttctccttggttttcatttccattctgggctaattgtctattaagtctcttaatctcttcttgtagctgttcctggtcttctcgctgtctctccatttgccgcatatgtgcttgccttaacaattccgttgcctgttgatgttcttggtattgtcgtacaagttcctgtctcatatcttccaactgttcttcattcaacattagttgtctagaagcatccatgcttgacactgaaatctcatcatgaatagactgtctaactataaatgttttatctttggagaacatttcttctgaaatagtcagcacacagtcctttgattctggtatatcatggggatcactatttgataataaaatttcctttccatgttctcctaactctttactaagtggtttaaattcttctttaaatttcacatccactgtctcaaaagtctgaaaaccaatttgatcctgtgataatttcatttcattaaaataatgttgttcttgctgacacacagcatgtgcttgctttgatgatgcagtattttcttttcccccagatattctagacagttcagtttgttgagcaaatgctatactcattgacacaataaccttagctacttcttcttctaattgttcttggtattgtttttcaagcaacttaacgatatttgtttcctctttcactccaaattcaccagaaaactctattgtaccatcaatattctttttcacacaacttccagggtacattgttctctgtgcatcagattctgtaattaccaccgaatcaacaggtaagcttggcggaaccgtggactcactaacagcttgaagcctcttctgtaaacagtggatctctgcctcatagttttgttcagtttctttcaactgttgctgcaaagaggatatgaggctttctaattcttgaacttgttcttcaagtttagttttttcaagatcttgcagagaagataacttgcttttatgattgacatcaatgtcttccaaattggtcatctgagaatggattgataaaaactctgtttcctcttttggaaggttttcttctccaaattcaagtttcataccatctgtctgctgtccccagatcttgcttagtcgtgtttgaagtaccaagagtttgttgtattcttctgttactttgttgagaagagtgtgcatattttcttgaaagtcttgaacttcatatctataatcttgtaattctggatcttcattttcagaaatgtaatcaccagaattctctttgtcttctgcatttacttcacattttaaagcaggagtataatattcaccaaggacactgcataaagtctgtaaaaaataagaacattcttcagacactgccttttgaagttttccaatgagcagatgtaaaggctttccttcatcacctgtttcttgtgttttcatagtctgtagttctaactggtgtattttctgaagttccttgatcttttcctcttgagcaaaaataagctcttctttaagactgcaaagagctttatctttttcattttccatatattcacgaacctgatccacatgagttgaataaaccagagagaggcaaatgcgttgggcttccatctgtagccttaaatcattctgttctgatttaagtacattgagttctttctgaagtttatcattttcacttggttgagttgctctaagtgatgattcctttgttacagatggtaagtgatccaaaatcaactgttcttgcttactttcttctccaacagtcatattttcaaaagaaactttatcttccaccattatttttgattcttcaccaaaacttttatttactttagaaactgatccttcagcacccctgcttgtcatggtcacaactccatctaataaagagcttacttgagtatcacatgactgtacattttctgccctgttgtggttaataatgatttctagctctctacatctcaatgaaacttgttctttctcttgctttaaagatttaacttcttcatttagaaaactaatctcaccatgtttctgtttcaattgttcagaaagatcagacagtctctgtgacagctctaatttctctcgcttggttacctcaagtttttccatgagttctgttgtatccttttcaacaacctcacccatttccaatgtttctgctacaaaagttttgtcttcatcaaagacagaacttttcattttcactgtagttggatttattctttgcaaatgaagctcttcattaagtgctttaagtttacttttatactctaattcctgtttatttttactgtcttctaaatcatcttttactttgagaaggcaagcatactcctcttgtaactcttgatagttaacttcaaagtttttttcagcaaatgaaaaagtgttcctttgcttttcaatctcttcatttagctgaatacattgttgtttgaggtcctcattttcctctataagtatttctatttctttttcccacacagagtctttggatttggacttaatggagtctaagaaaatcaatctttcttcttggctaacaggagtatgtattttcaacatgtcttcaagggttttcttttcatctttaagaatgctattctctgcttcaagttgtgcaaatttttcttgaagatcattctctttttccttcatctgtttttctaacaattctgttttaagttgtaattcttgaacttcttgttcaagtgtacccttttctttttcttcttgtctgagtatttcaatttctttttgaagttcattgatttgaagagtcatttcttctgactttgaatttacaagagactgctgtaaatcttttagctttgaaatttccaaaattaattgattctgcttagttatcaaattgtccttttcaaactgcatggtttctatcttttgactcatttcattctgtaaaccatctatctgctgtttatagtgaatgcctaaattatctttaagtttttcaatatttattcgatgttcaatttctaaatcttccttcagtttggaaagctcttcttcgtgactaaatagaagctgtgttctcagcctctctaattcagcttcttgtgattcagccattctgtctaacacagcattcttttctttttctaacatttcaagttttatcttgtaatttgtaacttctgcttcatgttttaattctagttcctttctggattcagatgcagaaacaatctcagctttcaaatcttccactgtactaagggacttatgtgcttcattaagtttactttcttgttcagctattgtctgtctagctctctgaatctgttcccttgaaaagctcaattcttcaacaaggtcttcaagctgtctctgtagagcacacttttcttctaaaattagtcctagttcttccttgagtttttccttttgagagttagtatcttgcaattttatattcagttcatttattgccacattcattaactttatctgatcttcattaactgtaatatttgaatatgaccttaaagcattctccatttctcccttatgccgtgttttcatttcctccatctgtgccatgtgttgtcttattaattcttgtttcatttgcactatctgctgcccatacatctcatccagctctgcccggagttgttctaactttctttgtgtttcttgttccattcgttgtactatatcagtttcgaactggctgtctttatgatttctcttctgaagttcttcgactgtccccattaactgttttatttcttcagaagactgtctttctttttgcttagaattagtcagctctaatttcatgttttttatttcttggttcttttgcacaatctgttcttgtaattctcctagtaatttatcagcagttgttaatttatcctttagctcaagagttttcttttcttcttctattatttttgtgtttaattcttcaatgattgtctccttttcctgtatttcttctttatttgagttttctacttttttatcttgttccatttcatatactttaattttctcttgcaagaaactaatttgcattgtgaagtcttctttctttttctgataatcttctaataagtggtcttgttcttcaagctgctgttgatgagtgaggatctgttgtttggcttgtagtaagtctgcagctgtgctactatgagtgctgtttctcagagtttcactagcctgtaattgctgaaattgaatctgtaatttttgactctgttctgtcaactctaaaaattctctcattgtctcatccttttctcttcttgcttgttgtaaattagcagtgagctgggttataatgccatctctttgtttaatggcagcttcaaattcttgtaactgctgcagtccttcagtcccataggtaaccctcatttcttccagctctctgtttagctcttcaatctcatgctgcttcccagccaactcactttccatcatctctagatgagtcggactgtcttgtgctccttgttcagaataagaatcatcaacaccaaattcttcttcccttaataaatttgtaggctttcctgttctcatcacaaaactgcaaccatttacctctgaactgcagtcatctgctgtggttgaaatttcactttccagttccacagagaagccctgctcatgactggttatttctccactatgtagagttctcattattgtagattcaggaatcacagttgattctactctctgagaactatttatgtacatttcattacactgtgattgatcaatattcaaatcatggtgtgctgacacatcatgtttactgcttgacgtttttctcttttttttctgcttcttggaaggactctgcccatccgactgagcttttctttgtcgaaactgggcaagcttggctttgccggcctccagcttcttctgtctctcctcgtcctccatggcctctgcaaggaaggcaggggaaaacaggggttgaggggtggttggggatagaaaggaaaggtcgatttggacggaggtgggacggcaagctccacggcctagagagccgattcggtccggcgctcccccgcccgaagtggaagcagtctccgcgctcactggcggatcgtcctcagccgcacgggaagcgccgtcaccgccgccgccgccgccatcttcgtctccacgta

SEQ ID NO: 14215 - RNA, 8620 nt, Homo sapiens
  source 1..8620: mol_type = other RNA
gctgggattacaggcatgagccaccgcgcccagcccatatacttaagctgacttttaagagattttgaatatatatgtaaaaatcaccatgactggctctatggcaaggtaggtgagactaatatttagagtttttttaaagtgctctcaaagttggatgttctatacctcatacatttttgaaaaatcttttggtcttcaaaatctgggtcttgtgaaatttggatgctcaaaacaaaacaagcctaggcaaaccaacaaactcagctatgataataaaagtttcctattactacaagatgcttgggtgtaaacaaatgatttcttgaaggaagagataaactactcaatgattcaaagtctctgaatcaggagtgaactgaagtgagatagggaaaagaggttttccttccatgaacagggaatccacctttattttaaagtatgacttgttttttgtttttgaacaaagaaaaaataatccttacaaagtattttaaatgggatagtttttttcgatgatacataaaagcacaatatagtagcagggataatggttacattaagtgcttaaagtaagtgcttcctccttaactccacccgatttgcatgccttaccactttcttttttttttttttttctttgagacagggtctcgctctgctgcccaggctggagtgctgcggcacggccttaccactttctgccatgcgctacttaggaatacgttctccagttaggctctgtagactcagagtaccttgcacactggtgctcattgtgcattttgtgtcatcagtccgctgaatgaacatagtaggaaatcatttttgggaggagtgggatctggggtgataaatcatattttcacttaaattatttaaagtcagtttctctgctggttacaagagtttaagctttggctaacttaataattagctcatgcactaaactggaagctttgattatcctaatgagtgtgaaagaatttcaaagaaaggggagctgtgggtctcgcactgtggtgctgccaagatgtggttaaactcagagcacctgactgtatagttccaagtcgtctttgcagtgcctctagccgagtgatataatctgttagggctctgtcaggatcgtaattctgaagctgagaacatgctaaagaaccaggattgaaatcagctggagtgcctgggtacctattctgaaatggtaaaggggacctaatatagtccagatctgatcttgagcgatacgtagtatgtcttggttctccatataactccagcccaccagaagaatgataaaatgagtcagtcttttctgcaccttgattcagtccaaagccatctctgttaatattgatggaaacagaacctgtgactcgatgccaccgtcgaaccaaaaatttcattctggaaattgcaatggatactctgacggccgaccgaaacctggtgaagccctttgggcgattggtgatcacctctagatccgtgaaagctggctgcccccccatccgggcaagcagggccaaggtggcatcttcacattcctggaacccacccagtaacagcagcaggtatttcttctggtaaatgagagcctttcgaaaactttctgccctcaagtatttaccataaattctctttaaagtgacatgttcagaatcagggctcagagtttgaagtaaagagtcatttcttagttcagctttcagtttgtatacttcagcctctgcccttttcaaagatttctggagagtcaatttttctctgttccatacttctttttcagaggcaatgatggcttcaatgttggcaccaccattcaatgaaaacctggaagaattatctctaccagctcctgtctgtcgataccacctgatctgctcttccagcttcataaccatgttccttaagtcattcttctcttcagtcagttgactgatatgccctgtcagctcagcattttgtctcagtagtctttcagtcaatgagccacaagaagtacttggggacaccaagctgggctcttcaccttgctggccagttaatttctgtagttgtaaaataatttcatcaatattttcctgaacccaaatgaaatcttcatcatctgctgtttcaaactgtagtctctcagaggctttctggggtagaacctgtagttttgaagctacacattgaagcttttgtctgatcatttctaattcatgattacagccggttcctcctccattcatttcaatcaatttagcgtagtttgattcttttgtttctccttctattttctgttgaagaacccaatttctagttctatcactggttaagctccacgtggttggctcattaaggttctgatacagaattcttctactttctcgtttttcttctcgttctagttcttgcttctggaattcctgcatgattccttgtagtcgctgtccttcaaggtctaacttataaacttgttgtcttttctcttccagctggcgctgaagatcttccactttggactggagctcatgcatttttttctgtccctcagtgttggcctcctgttctgtctgcagtgttttcctgtgaacctgcctatctttttccatttgctgtcgtgtttgcaaagaatccagtttatatttttcagtctcatttaacaattctactatgcgactgtgtttttcctctagctgtttctgcagctctttcagtaggtcctctgagggcaagggtggccgagactgtccagtaccatcactgctctgcagctgtgcgtgcaattcccgctccctatctagggtactactcatttcccgaattcgaactttctcagattcaagaagtacctgaagctctaagtttcgaccttgttcttctgacaactgggcatcatatagcattctctgtgattctattttttgctgggattcgttcagtagttgtttctgttgttccaaaagtagatttagctgaagattcctttgtttctgactctcaagtgaaaacttcagatcctcaagttcttctttatcccgttcttcactgcgtcccaacttggctttctctttctccaaagcccactggagctctcttgattttttctgttcacttgctaatgtgtcattaagcaaatgtacttcatctgtcttatctttaacttccaacctgaaagcctccaattcttttaggtgtttatgctgtgccttgagtgttgtttctagttccaatttagtttgtgcaagctcactcttcagttcagcaaccaccattttctcagaactcagctgctcctgcagttccgttgctctgtctttcatactgctgagctccacttgcatctccagcatttgagactgcttctgctgtatattatattccaagagttcttggcttggtttctcactctcttgttctcttttcagagtaattttcctaccattcatttgtgcatgcagtgcctgaatttcagataacaaactccttctatctgctttctggaggcattccatagctgcttgatattcaacaccctgttcttgtattctctgttccaaacagtttagtaaaccaactgcatctgtagtacctagagctgtcagctccgtccgaaatgctgctagtaaaacactacgctcttctaagaaaacttgttgaagggcaagcagtagttcacctcgccagtctgagaagctctcatgagattgagaactatcataaacctcggcttctctttgcagttgcatctttgtaattaaatcctttagagatgagattgtattgatgtaagcttttctctcttctagccaaggttctgaaacctgctgaatagaatggtcctctccatcactatagggagactcagtgagagaaagcacctgcatgccttcattatggacagctctcagtaatccctttattttctttggaaaggaatctgttgcactttcactttcttctcctcggccttctgatgctatgtcaaatccctgactgtgtgtaagataaattccctgaccccagtctgatccagaatcactggagcatatttctctagtctggtaagcatcagaatgtgctagctcaggaattgaggatccctctttacttctcagacactgtatcactgccttcaaggtaccacattcctctttcagtaactgaacggcaacatagtgttccctctttaaggtttcagtttctgaaatatgtctggattccatgtccaaaatttcagcagcatgtagttcttgcatcttctcaattttttcagtaaactgactgattatttcagtaacttcttctgaggaacattcactctgtaaattaatttgtattcctgcatttttaacaagaatttgtggagtctgattgctgctactgatcttcagagtcccatctgtctgggatgcaatgctcttactcagttttataggaagtggctcaaacatgcaggcctttttgctttcttgtacctcagtctcatcttctttttctaaaatggacaatttctcttttgcctctgcgaggtgatccctaacttggcttaagtctttctgaagagatgtcatatttgtttcttttaccaaaagctcttcttgaagtttttcagccttttctttataactggcaagttctgctttggtagccactgattcagctctaagagcctcgagttcattaaaaaatccactttcttcattgctatgaaatagctcagtagttgtcttgagaacttcaacatcttgagggcttcttttcttttctttctctctctgttttttctcattgccctccaatagcttctgtagttctagcagcttcttttctttttctaaaacatttttttctgcaatttctacttgttctttttctaaaatcaaactagtatgcatttcaacaacctggctttctaattctgatattctcaaggttaatgctgatatatctgaccccaactcatcttctcttagttgatttaaattctgaatatttgttctttcaggttctgatgaaattgtttgattatcttgacagaattttgcatattcctgaactgcctcaagttggatttgactgacaagagcagcagccactttttcttcaactattttctgtaggtttacaatcttcttttgaagcatttctgtttcaaactggccttgttcttgcatgtcttttatttgtttataacactgggtaagttctaagtcctttgcactaacagtgctctcaagttgtagcaaccttgtttccaaattaattatggaacctttgccattttcttcaaaagatttgaagtatgtctgattttctagggatttaagagcatcctctgtaaggactacttctagttcaggtttgtctttgctcagatgatctatagccacgttaacactattctctggtatgctttgaatcttttccacactttcacgttctctctttaagctgaataattcctgtgttagctgattcattttaaaattggtttctttaagtacatttttcatgaaggtcatttcttcattagcggtttctacttgctgttccaaggccagcttttcagctataaccacatccaattgatgttttaaactgtctgcttcttctgagagggaatgagcattcattgatgtcttctgtccaatatttgccaattcctgttgaagtttttcaatcacttcattgagctgctctatttcttcttctctatttctcttcacacattcttgatcactcatcaaacattctatttgggtttcaagatcccttatcagttcatttttttcttcaataaccttgttatctgttgtaattttaagttgctgctggagtttcgtaacttgttcatttaattggtcaatttctacctctttttcctgtattatttgagcaaatttcccaaatagcacatgttggtcttgagtagacatggcatcagattcctttatggcaagtcccagtttctccatgtcatccttaaataatttgttttcctgttcaagttcttgtaggcgggtagtagattcctttttctgtatttctaattgcatatgtaattgttgaacttcttcattcttattttccagttcttctctaaactgttctaattgctcttctaagtttgtaatctctttttcctttctgtctatggcatctcgttcagcctgcaattgtacttctagggacaattctggtttagcttctacagctccaaagtgttttcggtcctctaccttttgaaaagtatctgcactcacaagaagcgcctgctccagttctcttactctgaactccagtttctctatttcttcattcctttcttgtatatccctttgaagctgctctttagagagcaaaagctcactgcatttgtctgttttttctttcagatgatttgctaactgttcaacctctctagtttgatgttcactgataggctggaatcgaggaacaaccttaagttgctgttctagtttctgtatttcctgttggaatacatctctctcatgttctctgtcaatggcttgctcatctaaaaattttctcattttttctaactgcttttccaatgcttggttttgctgtcttaaatccattagttcagtatttttttcttgttccagctctataaacctactgacttgttcttccacatctatttctagagctttcacttgtttttgaaggtcatcacgtactttttcagcttgacattgtacttctagtttttccttcattaatttttctgtctcctgtagtaattctgctcctggtgctgcatcgactgcagcatctactagtcgttgttcaactgggcctgcctctgctttcatagcttccttttgtctggacagtaattctctttcttcttggatctgctgttgctctgcctccaattcttgcaacctgttacttgcacataacaactcctgctcaagacgatctattatatcagttttttcctgaatttgcctttcaaaaagagttttttcatctgcatagccatcaatgacgccctcagccttactgagctccacagctagctgttctctggccctggactcctcatgaaggcgctctcgaagttcctcttggcacttaagggactctgttgcttcttgtttctgtctaaatgactcacgcatcaactctgtctgtgtcactttcgcatgttcaagctgactgctagtttcacttatggcttctaggagtttttcaactgctgcttgtagtcgagagctaatgttcagcataagttcttcattttcagggtctatttcagttccagcaaaaccactcctcacaagtcgttgtgacagctctgttccttcctcagttacttttgaccacatgttaatgtcatttcttggcatatcacttccagaataagagggaatggattcatctgtaactcttgtatgttcctcatggacacatgactttacagatgcctctgcttctgacctccaaattaggctggcagatgactggcttttactagatctatctagaatcccaaggacatggcgaccaattgtttcttcaacagctgctgttgtctttacaacttctaagaggatcttcaaaagtctattattagctttctggagtgcatacactgtctttcttgtttgagttccatactgactgcgttccatactgatgatccaatggggaagccaaaatcttaggggccaaattcctccatgcaagctttcattagacaaaatctcaggaggcacatcttcaggttttctgtctaattccttttctttaaatgtttgttcttcaacttctccttggttttcatttccattctgtgtttgcgtactgctgttgcgcagctcacaacacagcttctctcttccagctaaagacagctgctttagtgcttccagctcctctaaaagcaccctctctctctctgaaaccaggttttcattatctatggaggatctctgggctaattgtctattaagtctcttaatctcttcttgtagctgttcctggtcttctcgctgtctctccatttgccgcatatgtgcttgccttaacaattccgttgcctgttgatgttcttggtattgtcgtacaagttcctgtctcatatcttccaactgttcttcattcaacattagttgtctagaagcatccatgcttgacactgaaatctcatcatgaatagactgtctaactataaatgttttatctttggagaacatttcttctgaaatagtcagcacacagtcctttgattctggtatatcatggggatcactatttgataataaaatttcctttccatgttctcctaactctttactaagtggtttaaattcttctttaaatttcacatccactgtctcaaaagtctgaaaaccaatttgatcctgtgataatttcatttcattaaaataatgttgttcttgctgacacacagcatgtgcttgctttgatgatgcagtattttcttttcccccagatattctagacagttcagtttgttgagcaaatgctatactcattgacacaataaccatcgataaaatctatgttctttttgaaggctcaaagggaatataaaccaagataatcttccagataagctataagccta

SEQ ID NO: 14216 - RNA, 13018 nt, Homo sapiens
  source 1..13018: mol_type = other RNA
gctgggattacaggcatgagccaccgcgcccagcccatatacttaagctgacttttaagagattttgaatatatatgtaaaaatcaccatgactggctctatggcaaggtaggtgagactaatatttagagtttttttaaagtgctctcaaagttggatgttctatacctcatacatttttgaaaaatcttttggtcttcaaaatctgggtcttgtgaaatttggatgctcaaaacaaaacaagcctaggcaaaccaacaaactcagctatgataataaaagtttcctattactacaagatgcttgggtgtaaacaaatgatttcttgaaggaagagataaactactcaatgattcaaagtctctgaatcaggagtgaactgaagtgagatagggaaaagaggttttccttccatgaacagggaatccacctttattttaaagtatgacttgttttttgtttttgaacaaagaaaaaataatccttacaaagtattttaaatgggatagtttttttcgatgatacataaaagcacaatatagtagcagggataatggttacattaagtgcttaaagtaagtgcttcctccttaactccacccgatttgcatgccttaccactttcttttttttttttttttctttgagacagggtctcgctctgctgcccaggctggagtgctgcggcacggccttaccactttctgccatgcgctacttaggaatacgttctccagttaggctctgtagactcagagtaccttgcacactggtgctcattgtgcattttgtgtcatcagtccgctgaatgaacatagtaggaaatcatttttgggaggagtgggatctggggtgataaatcatattttcacttaaattatttaaagtcagtttctctgctggttacaagagtttaagctttggctaacttaataattagctcatgcactaaactggaagctttgattatcctaatgagtgtgaaagaatttcaaagaaaggggagctgtgggtctcgcactgtggtgctgccaagatgtggttaaactcagagcacctgactgtatagttccaagtcgtctttgcagtgcctctagccgagtgatataatctgttagggctctgtcaggatcgtaattctgaagctgagaacatgctaaagaaccaggattgaaatcagctggagtgcctgggtacctattctgaaatggtaaaggggacctaatatagtccagatctgatcttgagcgatacgtagtatgtcttggttctccatataactccagcccaccagaagaatgataaaatgagtcagtcttttctgcaccttgattcagtccaaagccatctctgttaatattgatggaaacagaacctgtgactcgatgccaccgtcgaaccaaaaatttcattctggaaattgcaatggatactctgacggccgaccgaaacctggtgaagccctttgggcgattggtgatcacctctagatccgtgaaagctggctgcccccccatccgggcaagcagggccaaggtggcatcttcacattcctggaacccacccagtaacagcagcaggtatttcttctggtaaatgagagcctttcgaaaactttctgccctcaagtatttaccataaattctctttaaagtgacatgttcagaatcagggctcagagtttgaagtaaagagtcatttcttagttcagctttcagtttgtatacttcagcctctgcccttttcaaagatttctggagagtcaatttttctctgttccatacttctttttcagaggcaatgatggcttcaatgttggcaccaccattcaatgaaaacctggaagaattatctctaccagctcctgtctgtcgataccacctgatctgctcttccagcttcataaccatgttccttaagtcattcttctcttcagtcagttgactgatatgccctgtcagctcagcattttgtctcagtagtctttcagtcaatgagccacaagaagtacttggggacaccaagctgggctcttcaccttgctggccagttaatttctgtagttgtaaaataatttcatcaatattttcctgaacccaaatgaaatcttcatcatctgctgtttcaaactgtagtctctcagaggctttctggggtagaacctgtagttttgaagctacacattgaagcttttgtctgatcatttctaattcatgattacagccggttcctcctccattcatttcaatcaatttagcgtagtttgattcttttgtttctccttctattttctgttgaagaacccaatttctagttctatcactggttaagctccacgtggttggctcattaaggttctgatacagaattcttctactttctcgtttttcttctcgttctagttcttgcttctggaattcctgcatgattccttgtagtcgctgtccttcaaggtctaacttataaacttgttgtcttttctcttccagctggcgctgaagatcttccactttggactggagctcatgcatttttttctgtccctcagtgttggcctcctgttctgtctgcagtgttttcctgtgaacctgcctatctttttccatttgctgtcgtgtttgcaaagaatccagtttatatttttcagtctcatttaacaattctactatgcgactgtgtttttcctctagctgtttctgcagctctttcagtaggtcctctgagggcaagggtggccgagactgtccagtaccatcactgctctgcagctgtgcgtgcaattcccgctccctatctagggtactactcatttcccgaattcgaactttctcagattcaagaagtacctgaagctctaagtttcgaccttgttcttctgacaactgggcatcatatagcattctctgtgattctattttttgctgggattcgttcagtagttgtttctgttgttccaaaagtagatttagctgaagattcctttgtttctgactctcaagtgaaaacttcagatcctcaagttcttctttatcccgttcttcactgcgtcccaacttggctttctctttctccaaagcccactggagctctcttgattttttctgttcacttgctaatgtgtcattaagcaaatgtacttcatctgtcttatctttaacttccaacctgaaagcctccaattcttttaggtgtttatgctgtgccttgagtgttgtttctagttccaatttagtttgtgcaagctcactcttcagttcagcaaccaccattttctcagaactcagctgctcctgcagttccgttgctctgtctttcatactgctgagctccacttgcatctccagcatttgagactgcttctgctgtatattatattccaagagttcttggcttggtttctcactctcttgttctcttttcagagtaattttcctaccattcatttgtgcatgcagtgcctgaatttcagataacaaactccttctatctgctttctggaggcattccatagctgcttgatattcaacaccctgttcttgtattctctgttccaaacagtttagtaaaccaactgcatctgtagtacctagagctgtcagctccgtccgaaatgctgctagtaaaacactacgctcttctaagaaaacttgttgaagggcaagcagtagttcacctcgccagtctgagaagctctcatgagattgagaactatcataaacctcggcttctctttgcagttgcatctttgtaattaaatcctttagagatgagattgtattgatgtaagcttttctctcttctagccaaggttctgaaacctgctgaatagaatggtcctctccatcactatagggagactcagtgagagaaagcacctgcatgccttcattatggacagctctcagtaatccctttattttctttggaaaggaatctgttgcactttcactttcttctcctcggccttctgatgctatgtcaaatccctgactgtgtgtaagataaattccctgaccccagtctgatccagaatcactggagcatatttctctagtctggtaagcatcagaatgtgctagctcaggaattgaggatccctctttacttctcagacactgtatcactgccttcaaggtaccacattcctctttcagtaactgaacggcaacatagtgttccctctttaaggtttcagtttctgaaatatgtctggattccatgtccaaaatttcagcagcatgtagttcttgcatcttctcaattttttcagtaaactgactgattatttcagtaacttcttctgaggaacattcactctgtaaattaatttgtattcctgcatttttaacaagaatttgtggagtctgattgctgctactgatcttcagagtcccatctgtctgggatgcaatgctcttactcagttttataggaagtggctcaaacatgcaggcctttttgctttcttgtacctcagtctcatcttctttttctaaaatggacaatttctcttttgcctctgcgaggtgatccctaacttggcttaagtctttctgaagagatgtcatatttgtttcttttaccaaaagctcttcttgaagtttttcagccttttctttataactggcaagttctgctttggtagccactgattcagctctaagagcctcgagttcattaaaaaatccactttcttcattgctatgaaatagctcagtagttgtcttgagaacttcaacatcttgagggcttcttttcttttctttctctctctgttttttctcattgccctccaatagcttctgtagttctagcagcttcttttctttttctaaaacatttttttctgcaatttctacttgttctttttctaaaatcaaactagtatgcatttcaacaacctggctttctaattctgatattctcaaggttaatgctgatatatctgaccccaactcatcttctcttagttgatttaaattctgaatatttgttctttcaggttctgatgaaattgtttgattatcttgacagaattttgcatattcctgaactgcctcaagttggatttgactgacaagagcagcagccactttttcttcaactattttctgtaggtttacaatcttcttttgaagcatttctgtttcaaactggccttgttcttgcatgtcttttatttgtttataacactgggtaagttctaagtcctttgcactaacagtgctctcaagttgtagcaaccttgtttccaaattaattatggaacctttgccattttcttcaaaagatttgaagtatgtctgattttctagggatttaagagcatcctctgtaaggactacttctagttcaggtttgtctttgctcagatgatctatagccacgttaacactattctctggtatgctttgaatcttttccacactttcacgttctctctttaagctgaataattcctgtgttagctgattcattttaaaattggtttctttaagtacatttttcatgaaggtcatttcttcattagcggtttctacttgctgttccaaggccagcttttcagctataaccacatccaattgatgttttaaactgtctgcttcttctgagagggaatgagcattcattgatgtcttctgtccaatatttgccaattcctgttgaagtttttcaatcacttcattgagctgctctatttcttcttctctatttctcttcacacattcttgatcactcatcaaacattctatttgggtttcaagatcccttatcagttcatttttttcttcaataaccttgttatctgttgtaattttaagttgctgctggagtttcgtaacttgttcatttaattggtcaatttctacctctttttcctgtattatttgagcaaatttcccaaatagcacatgttggtcttgagtagacatggcatcagattcctttatggcaagtcccagtttctccatgtcatccttaaataatttgttttcctgttcaagttcttgtaggcgggtagtagattcctttttctgtatttctaattgcatatgtaattgttgaacttcttcattcttattttccagttcttctctaaactgttctaattgctcttctaagtttgtaatctctttttcctttctgtctatggcatctcgttcagcctgcaattgtacttctagggacaattctggtttagcttctacagctccaaagtgttttcggtcctctaccttttgaaaagtatctgcactcacaagaagcgcctgctccagttctcttactctgaactccagtttctctatttcttcattcctttcttgtatatccctttgaagctgctctttagagagcaaaagctcactgcatttgtctgttttttctttcagatgatttgctaactgttcaacctctctagtttgatgttcactgataggctggaatcgaggaacaaccttaagttgctgttctagtttctgtatttcctgttggaatacatctctctcatgttctctgtcaatggcttgctcatctaaaaattttctcattttttctaactgcttttccaatgcttggttttgctgtcttaaatccattagttcagtatttttttcttgttccagctctataaacctactgacttgttcttccacatctatttctagagctttcacttgtttttgaaggtcatcacgtactttttcagcttgacattgtacttctagtttttccttcattaatttttctgtctcctgtagtaattctgctcctggtgctgcatcgactgcagcatctactagtcgttgttcaactgggcctgcctctgctttcatagcttccttttgtctggacagtaattctctttcttcttggatctgctgttgctctgcctccaattcttgcaacctgttacttgcacataacaactcctgctcaagacgatctattatatcagttttttcctgaatttgcctttcaaaaagagttttttcatctgcatagccatcaatgacgccctcagccttactgagctccacagctagctgttctctggccctggactcctcatgaaggcgctctcgaagttcctcttggcacttaagggactctgttgcttcttgtttctgtctaaatgactcacgcatcaactctgtctgtgtcactttcgcatgttcaagctgactgctagtttcacttatggcttctaggagtttttcaactgctgcttgtagtcgagagctaatgttcagcataagttcttcattttcagggtctatttcagttccagcaaaaccactcctcacaagtcgttgtgacagctctgttccttcctcagttacttttgaccacatgttaatgtcatttcttggcatatcacttccagaataagagggaatggattcatctgtaactcttgtatgttcctcatggacacatgactttacagatgcctctgcttctgacctccaaattaggctggcagatgactggcttttactagatctatctagaatcccaaggacatggcgaccaattgtttcttcaacagctgctgttgtctttacaacttctaagaggatcttcaaaagtctattattagctttctggagtgcatacactgtctttcttgtttgagttccatactgactgcgttccatactgatgatccaatggggaagccaaaatcttaggggccaaattcctccatgcaagctttcattagacaaaatctcaggaggcacatcttcaggttttctgtctaattccttttctttaaatgtttgttcttcaacttctccttggttttcatttccattctgtgtttgcgtactgctgttgcgcagctcacaacacagcttctctcttccagctaaagacagctgctttagtgcttccagctcctctaaaagcaccctctctctctctgaaaccaggttttcattatctatggaggatctctgggctaattgtctattaagtctcttaatctcttcttgtagctgttcctggtcttctcgctgtctctccatttgccgcatatgtgcttgccttaacaattccgttgcctgttgatgttcttggtattgtcgtacaagttcctgtctcatatcttccaactgttcttcattcaacattagttgtctagaagcatccatgcttgacactgaaatctcatcatgaatagactgtctaactataaatgttttatctttggagaacatttcttctgaaatagtcagcacacagtcctttgattctggtatatcatggggatcactatttgataataaaatttcctttccatgttctcctaactctttactaagtggtttaaattcttctttaaatttcacatccactgtctcaaaagtctgaaaaccaatttgatcctgtgataatttcatttcattaaaataatgttgttcttgctgacacacagcatgtgcttgctttgatgatgcagtattttcttttcccccagatattctagacagttcagtttgttgagcaaatgctatactcattgacacaataacctctattgtaccatcaatattctttttcacacaacttccagggtacattgttctctgtgcatcagattctgtaattaccaccgaatcaacaggtaagcttggcggaaccgtggactcactaacagcttgaagcctcttctgtaaacagtggatctctgcctcatagttttgttcagtttctttcaactgttgctgcaaagaggatatgaggctttctaattcttgaacttgttcttcaagtttagttttttcaagatcttgcagagaagataacttgcttttatgattgacatcaatgtcttccaaattggtcatctgagaatggattgataaaaactctgtttcctcttttggaaggttttcttctccaaattcaagtttcataccatctgtctgctgtccccagatcttgcttagtcgtgtttgaagtaccaagagtttgttgtattcttctgttactttgttgagaagagtgtgcatattttcttgaaagtcttgaacttcatatctataatcttgtaattctggatcttcattttcagaaatgtaatcaccagaattctctttgtcttctgcatttacttcacattttaaagcaggagtataatattcaccaaggacactgcataaagtctgtaaaaaataagaacattcttcagacactgccttttgaagttttccaatgagcagatgtaaaggctttccttcatcacctgtttcttgtgttttcatagtctgtagttctaactggtgtattttctgaagttccttgatcttttcctcttgagcaaaaataagctcttctttaagactgcaaagagctttatctttttcattttccatatattcacgaacctgatccacatgagttgaataaaccagagagaggcaaatgcgttgggcttccatctgtagccttaaatcattctgttctgatttaagtacattgagttctttctgaagtttatcattttcacttggttgagttgctctaagtgatgattcctttgttacagatggtaagtgatccaaaatcaactgttcttgcttactttcttctccaacagtcatattttcaaaagaaactttatcttccaccattatttttgattcttcaccaaaacttttatttactttagaaactgatccttcagcacccctgcttgtcatggtcacaactccatctaataaagagcttacttgagtatcacatgactgtacattttctgccctgttgtggttaataatgatttctagctctctacatctcaatgaaacttgttctttctcttgctttaaagatttaacttcttcatttagaaaactaatctcaccatgtttctgtttcaattgttcagaaagatcagacagtctctgtgacagctctaatttctctcgcttggttacctcaagtttttccatgagttctgttgtatccttttcaacaacctcacccatttccaatgtttctgctacaaaagttttgtcttcatcaaagacagaacttttcattttcactgtagttggatttattctttgcaaatgaagctcttcattaagtgctttaagtttacttttatactctaattcctgtttatttttactgtcttctaaatcatcttttactttgagaaggcaagcatactcctcttgtaactcttgatagttaacttcaaagtttttttcagcaaatgaaaaagtgttcctttgcttttcaatctcttcatttagctgaatacattgttgtttgaggtcctcattttcctctataagtatttctatttctttttcccacacagagtctttggatttggacttaatggagtctaagaaaatcaatctttcttcttggctaacaggagtatgtattttcaacatgtcttcaagggttttcttttcatctttaagaatgctattctctgcttcaagttgtgcaaatttttcttgaagatcattctctttttccttcatctgtttttctaacaattctgttttaagttgtaattcttgaacttcttgttcaagtgtacccttttctttttcttcttgtctgagtatttcaatttctttttgaagttcattgatttgaagagtcatttcttctgactttgaatttacaagagactgctgtaaatcttttagctttgaaatttccaaaattaattgattctgcttagttatcaaattgtccttttcaaactgcatggtttctatcttttgactcatttcattctgtaaaccatctatctgctgtttatagtgaatgcctaaattatctttaagtttttcaatatttattcgatgttcaatttctaaatcttccttcagtttggaaagctcttcttcgtgactaaatagaagctgtgttctcagcctctctaattcagcttcttgtgattcagccattctgtctaacacagcattcttttctttttctaacatttcaagttttatcttgtaatttgtaacttctgcttcatgttttaattctagttcctttctggattcagatgcagaaacaatctcagctttcaaatcttccactgtactaagggacttatgtgcttcattaagtttactttcttgttcagctattgtctgtctagctctctgaatctgttcccttgaaaagctcaattcttcaacaaggtcttcaagctgtctctgtagagcacacttttcttctaaaattagtcctagttcttccttgagtttttccttttgagagttagtatcttgcaattttatattcagttcatttattgccacattcattaactttatctgatcttcattaactgtaatatttgaatatgaccttaaagcattctccatttctcccttatgccgtgttttcatttcctccatctgtgccatgtgttgtcttattaattcttgtttcatttgcactatctgctgcccatacatctcatccagctctgcccggagttgttctaactttctttgtgtttcttgttccattcgttgtactatatcagtttcgaactggctgtctttatgatttctcttctgaagttcttcgactgtccccattaactgttttatttcttcagaagactgtctttctttttgcttagaattagtcagctctaatttcatgttttttatttcttggttcttttgcacaatctgttcttgtaattctcctagtaatttatcagcagttgttaatttatcctttagctcaagagttttcttttcttcttctattatttttgtgtttaattcttcaatgattgtctccttttcctgtatttcttctttatttgagttttctacttttttatcttgttccatttcatatactttaattttctcttgcaagaaactaatttgcattgtgaagtcttctttctttttctgataatcttctaataagtggtcttgttcttcaagctgctgttgatgagtgaggatctgttgtttggcttgtagtaagtctgcagctgtgctactatgagtgctgtttctcagagtttcactagcctgtaattgctgaaattgaatctgtaatttttgactctgttctgtcaactctaaaaattctctcattgtctcatccttttctcttcttgcttgttgtaaattagcagtgagctgggttataatgccatctctttgtttaatggcagcttcaaattcttgtaactgctgcagtccttcagtcccataggtaaccctcatttcttccagctctctgtttagctcttcaatctcatgctgcttcccagccaactcactttccatcatctctagatgagtcggactgtcttgtgctccttgttcagaataagaatcatcaacaccaaattcttcttcccttaataaatttgtaggctttcctgttctcatcacaaaactgcaaccatttacctctgaactgcagtcatctgctgtggttgaaatttcactttccagttccacagagaagccctgctcatgactggttatttctccactatgtagagttctcattattgtagattcaggaatcacagttgattctactctctgagaactatttatgtacatttcattacactgtgattgatcaatattcaaatcatggtgtgctgacacatcatgtttactgcttgacgtttttctcttttttttctgcttcttggaaggactctgcccatccgactgagcttttctttgtcgaaactgggcaagcttggctttgccggcctccagcttcttctgtctctcctcgtcctccatggcctctgcaaggaaggcaggggaaaacaggggttgaggggtggttggggatagaaaggaaaggtcgatttggacggaggtgggacggcaagctccacggcctagagagccgattcggtccggcgctcccccgcccgaagtggaagcagtctccgcgctcactggcggatcgtcctcagccgcacgggaagcgccgtcaccgccgccgccgccgccatcttcgtctccacgta

SEQ ID NO: 14217 - RNA, 12700 nt, Homo sapiens
  source 1..12700: mol_type = other RNA
gctgggattacaggcatgagccaccgcgcccagcccatatacttaagctgacttttaagagattttgaatatatatgtaaaaatcaccatgactggctctatggcaaggtaggtgagactaatatttagagtttttttaaagtgctctcaaagttggatgttctatacctcatacatttttgaaaaatcttttggtcttcaaaatctgggtcttgtgaaatttggatgctcaaaacaaaacaagcctaggcaaaccaacaaactcagctatgataataaaagtttcctattactacaagatgcttgggtgtaaacaaatgatttcttgaaggaagagataaactactcaatgattcaaagtctctgaatcaggagtgaactgaagtgagatagggaaaagaggttttccttccatgaacagggaatccacctttattttaaagtatgacttgttttttgtttttgaacaaagaaaaaataatccttacaaagtattttaaatgggatagtttttttcgatgatacataaaagcacaatatagtagcagggataatggttacattaagtgcttaaagtaagtgcttcctccttaactccacccgatttgcatgccttaccactttcttttttttttttttttctttgagacagggtctcgctctgctgcccaggctggagtgctgcggcacggccttaccactttctgccatgcgctacttaggaatacgttctccagttaggctctgtagactcagagtaccttgcacactggtgctcattgtgcattttgtgtcatcagtccgctgaatgaacatagtaggaaatcatttttgggaggagtgggatctggggtgataaatcatattttcacttaaattatttaaagtcagtttctctgctggttacaagagtttaagctttggctaacttaataattagctcatgcactaaactggaagctttgattatcctaatgagtgtgaaagaatttcaaagaaaggggagctgtgggtctcgcactgtggtgctgccaagatgtggttaaactcagagcacctgactgtatagttccaagtcgtctttgcagtgcctctagccgagtgatataatctgttagggctctgtcaggatcgtaattctgaagctgagaacatgctaaagaaccaggattgaaatcagctggagtgcctgggtacctattctgaaatggtaaaggggacctaatatagtccagatctgatcttgagcgatacgtagtatgtcttggttctccatataactccagcccaccagaagaatgataaaatgagtcagtcttttctgcaccttgattcagtccaaagccatctctgttaatattgatggaaacagaacctgtgactcgatgccaccgtcgaaccaaaaatttcattctggaaattgcaatggatactctgacggccgaccgaaacctggtgaagccctttgggcgattggtgatcacctctagatccgtgaaagctggctgcccccccatccgggcaagcagggccaaggtggcatcttcacattcctggaacccacccagtaacagcagcaggtatttcttctggtaaatgagagcctttcgaaaactttctgccctcaagtatttaccataaattctctttaaagtgacatgttcagaatcagggctcagagtttgaagtaaagagtcatttcttagttcagctttcagtttgtatacttcagcctctgcccttttcaaagatttctggagagtcaatttttctctgttccatacttctttttcagaggcaatgatggcttcaatgttggcaccaccattcaatgaaaacctggaagaattatctctaccagctcctgtctgtcgataccacctgatctgctcttccagcttcataaccatgttccttaagtcattcttctcttcagtcagttgactgatatgccctgtcagctcagcattttgtctcagtagtctttcagtcaatgagccacaagaagtacttggggacaccaagctgggctcttcaccttgctggccagttaatttctgtagttgtaaaataatttcatcaatattttcctgaacccaaatgaaatcttcatcatctgctgtttcaaactgtagtctctcagaggctttctggggtagaacctgtagttttgaagctacacattgaagcttttgtctgatcatttctaattcatgattacagccggttcctcctccattcatttcaatcaatttagcgtagtttgattcttttgtttctccttctattttctgttgaagaacccaatttctagttctatcactggttaagctccacgtggttggctcattaaggttctgatacagaattcttctactttctcgtttttcttctcgttctagttcttgcttctggaattcctgcatgattccttgtagtcgctgtccttcaaggtctaacttataaacttgttgtcttttctcttccagctggcgctgaagatcttccactttggactggagctcatgcatttttttctgtccctcagtgttggcctcctgttctgtctgcagtgttttcctgtgaacctgcctatctttttccatttgctgtcgtgtttgcaaagaatccagtttatatttttcagtctcatttaacaattctactatgcgactgtgtttttcctctagctgtttctgcagctctttcagtaggtcctctgagggcaagggtggccgagactgtccagtaccatcactgctctgcagctgtgcgtgcaattcccgctccctatctagggtactactcatttcccgaattcgaactttctcagattcaagaagtacctgaagctctaagtttcgaccttgttcttctgacaactgggcatcatatagcattctctgtgattctattttttgctgggattcgttcagtagttgtttctgttgttccaaaagtagatttagctgaagattcctttgtttctgactctcaagtgaaaacttcagatcctcaagttcttctttatcccgttcttcactgcgtcccaacttggctttctctttctccaaagcccactggagctctcttgattttttctgttcacttgctaatgtgtcattaagcaaatgtacttcatctgtcttatctttaacttccaacctgaaagcctccaattcttttaggtgtttatgctgtgccttgagtgttgtttctagttccaatttagtttgtgcaagctcactcttcagttcagcaaccaccattttctcagaactcagctgctcctgcagttccgttgctctgtctttcatactgctgagctccacttgcatctccagcatttgagactgcttctgctgtatattatattccaagagttcttggcttggtttctcactctcttgttctcttttcagagtaattttcctaccattcatttgtgcatgcagtgcctgaatttcagataacaaactccttctatctgctttctggaggcattccatagctgcttgatattcaacaccctgttcttgtattctctgttccaaacagtttagtaaaccaactgcatctgtagtacctagagctgtcagctccgtccgaaatgctgctagtaaaacactacgctcttctaagaaaacttgttgaagggcaagcagtagttcacctcgccagtctgagaagctctcatgagattgagaactatcataaacctcggcttctctttgcagttgcatctttgtaattaaatcctttagagatgagattgtattgatgtaagcttttctctcttctagccaaggttctgaaacctgctgaatagaatggtcctctccatcactatagggagactcagtgagagaaagcacctgcatgccttcattatggacagctctcagtaatccctttattttctttggaaaggaatctgttgcactttcactttcttctcctcggccttctgatgctatgtcaaatccctgactgtgtgtaagataaattccctgaccccagtctgatccagaatcactggagcatatttctctagtctggtaagcatcagaatgtgctagctcaggaattgaggatccctctttacttctcagacactgtatcactgccttcaaggtaccacattcctctttcagtaactgaacggcaacatagtgttccctctttaaggtttcagtttctgaaatatgtctggattccatgtccaaaatttcagcagcatgtagttcttgcatcttctcaattttttcagtaaactgactgattatttcagtaacttcttctgaggaacattcactctgtaaattaatttgtattcctgcatttttaacaagaatttgtggagtctgattgctgctactgatcttcagagtcccatctgtctgggatgcaatgctcttactcagttttataggaagtggctcaaacatgcaggcctttttgctttcttgtacctcagtctcatcttctttttctaaaatggacaatttctcttttgcctctgcgaggtgatccctaacttggcttaagtctttctgaagagatgtcatatttgtttcttttaccaaaagctcttcttgaagtttttcagccttttctttataactggcaagttctgctttggtagccactgattcagctctaagagcctcgagttcattaaaaaatccactttcttcattgctatgaaatagctcagtagttgtcttgagaacttcaacatcttgagggcttcttttcttttctttctctctctgttttttctcattgccctccaatagcttctgtagttctagcagcttcttttctttttctaaaacatttttttctgcaatttctacttgttctttttctaaaatcaaactagtatgcatttcaacaacctggctttctaattctgatattctcaaggttaatgctgatatatctgaccccaactcatcttctcttagttgatttaaattctgaatatttgttctttcaggttctgatgaaattgtttgattatcttgacagaattttgcatattcctgaactgcctcaagttggatttgactgacaagagcagcagccactttttcttcaactattttctgtaggtttacaatcttcttttgaagcatttctgtttcaaactggccttgttcttgcatgtcttttatttgtttataacactgggtaagttctaagtcctttgcactaacagtgctctcaagttgtagcaaccttgtttccaaattaattatggaacctttgccattttcttcaaaagatttgaagtatgtctgattttctagggatttaagagcatcctctgtaaggactacttctagttcaggtttgtctttgctcagatgatctatagccacgttaacactattctctggtatgctttgaatcttttccacactttcacgttctctctttaagctgaataattcctgtgttagctgattcattttaaaattggtttctttaagtacatttttcatgaaggtcatttcttcattagcggtttctacttgctgttccaaggccagcttttcagctataaccacatccaattgatgttttaaactgtctgcttcttctgagagggaatgagcattcattgatgtcttctgtccaatatttgccaattcctgttgaagtttttcaatcacttcattgagctgctctatttcttcttctctatttctcttcacacattcttgatcactcatcaaacattctatttgggtttcaagatcccttatcagttcatttttttcttcaataaccttgttatctgttgtaattttaagttgctgctggagtttcgtaacttgttcatttaattggtcaatttctacctctttttcctgtattatttgagcaaatttcccaaatagcacatgttggtcttgagtagacatggcatcagattcctttatggcaagtcccagtttctccatgtcatccttaaataatttgttttcctgttcaagttcttgtaggcgggtagtagattcctttttctgtatttctaattgcatatgtaattgttgaacttcttcattcttattttccagttcttctctaaactgttctaattgctcttctaagtttgtaatctctttttcctttctgtctatggcatctcgttcagcctgcaattgtacttctagggacaattctggtttagcttctacagctccaaagtgttttcggtcctctaccttttgaaaagtatctgcactcacaagaagcgcctgctccagttctcttactctgaactccagtttctctatttcttcattcctttcttgtatatccctttgaagctgctctttagagagcaaaagctcactgcatttgtctgttttttctttcagatgatttgctaactgttcaacctctctagtttgatgttcactgataggctggaatcgaggaacaaccttaagttgctgttctagtttctgtatttcctgttggaatacatctctctcatgttctctgtcaatggcttgctcatctaaaaattttctcattttttctaactgcttttccaatgcttggttttgctgtcttaaatccattagttcagtatttttttcttgttccagctctataaacctactgacttgttcttccacatctatttctagagctttcacttgtttttgaaggtcatcacgtactttttcagcttgacattgtacttctagtttttccttcattaatttttctgtctcctgtagtaattctgctcctggtgctgcatcgactgcagcatctactagtcgttgttcaactgggcctgcctctgctttcatagcttccttttgtctggacagtaattctctttcttcttggatctgctgttgctctgcctccaattcttgcaacctgttacttgcacataacaactcctgctcaagacgatctattatatcagttttttcctgaatttgcctttcaaaaagagttttttcatctgcatagccatcaatgacgccctcagccttactgagctccacagctagctgttctctggccctggactcctcatgaaggcgctctcgaagttcctcttggcacttaagggactctgttgcttcttgtttctgtctaaatgactcacgcatcaactctgtctgtgtcactttcgcatgttcaagctgactgctagtttcacttatggcttctaggagtttttcaactgctgcttgtagtcgagagctaatgttcagcataagttcttcattttcagggtctatttcagttccagcaaaaccactcctcacaagtcgttgtgacagctctgttccttcctcagttacttttgaccacatgttaatgtcatttcttggcatatcacttccagaataagagggaatggattcatctgtaactcttgtatgttcctcatggacacatgactttacagatgcctctgcttctgacctccaaattaggctggcagatgactggcttttactagatctatctagaatcccaaggacatggcgaccaattgtttcttcaacagctgctgttgtctttacaacttctaagaggatcttcaaaagtctattattagctttctggagtgcatacactgtctttcttgtttgagttccatactgactgcgttccatactgatgatccaatggggaagccaaaatcttaggggccaaattcctccatgcaagctttcattagacaaaatctcaggaggcacatcttcaggttttctgtctaattccttttctttaaatgtttgttcttcaacttctccttggttttcatttccattctgtgtttgcgtactgctgttgcgcagctcacaacacagcttctctcttccagctaaagacagctgctttagtgcttccagctcctctaaaagcaccctctctctctctgaaaccaggttttcattatctatggaggatctctgggctaattgtctattaagtctcttaatctcttcttgtagctgttcctggtcttctcgctgtctctccatttgccgcatatgtgcttgccttaacaattccgttgcctgttgatgttcttggtattgtcgtacaagttcctgtctcatatcttccaactgttcttcattcaacattagttgtctagaagcatccatgcttgacactgaaatctcatcatgaatagactgtctaactataaatgttttatctttggagaacatttcttctgaaatagtcagcacacagtcctttgattctggtatatcatggggatcactatttgataataaaatttcctttccatgttctcctaactctttactaagtggtttaaattcttctttaaatttcacatccactgtctcaaaagtctgaaaaccaatttgatcctgtgataatttcatttcattaaaataatgttgttcttgctgacacacagcatgtgcttgctttgatgatgcagtattttcttttcccccagatattctagacagttcagtttgttgagcaaatgctatactcattgacacaataaccttagctacttcttcttctaattgttcttggtattgtttttcaagcaacttaacgatatttgtttcctctttcactccaaattcaccagaaaactctattgtaccatcaatattctttttcacacaacttccagggtacattgttctctgtgcatcagattctgtaattaccaccgaatcaacaggtaagcttggcggaaccgtggactcactaacagcttgaagcctcttctgtaaacagtggatctctgcctcatagttttgttcagtttctttcaactgttgctgcaaagaggatatgaggctttctaattcttgaacttgttcttcaagtttagttttttcaagatcttgcagagaagataacttgcttttatgattgacatcaatgtcttccaaattggtcatctgagaatggattgataaaaactctgtttcctcttttggaaggttttcttctccaaattcaagtttcataccatctgtctgctgtccccagatcttgcttagtcgtgtttgaagtaccaagagtttgttgtattcttctgttactttgttgagaagagtgtgcatattttcttgaaagtcttgaacttcatatctataatcttgtaattctggatcttcattttcagaaatgtaatcaccagaattctctttgtcttctgcatttacttcacattttaaagcaggagtataatattcaccaaggacactgcataaagtctgtaaaaaataagaacattcttcagacactgccttttgaagttttccaatgagcagatgtaaaggctttccttcatcacctgtttcttgtgttttcatagtctgtagttctaactggtgtattttctgaagttccttgatcttttcctcttgagcaaaaataagctcttctttaagactgcaaagagctttatctttttcattttccatatattcacgaacctgatccacatgagttgaataaaccagagagaggcaaatgcgttgggcttccatctgtagccttaaatcattctgttctgatttaagtacattgagttctttctgaagtttatcattttcacttggttgagttgctctaagtgatgattcctttgttacagatggtaagtgatccaaaatcaactgttcttgcttactttcttctccaacagtcatattttcaaaagaaactttatcttccaccattatttttgattcttcaccaaaacttttatttactttagaaactgatccttcagcacccctgcttgtcatggtcacaactccatctaataaagagcttacttgagtatcacatgactgtacattttctgccctgttgtggttaataatgatttctagctctctacatctcaatgaaacttgttctttctcttgctttaaagatttaacttcttcatttagaaaactaatctcaccatgtttctgtttcaattgttcagaaagatcagacagtctctgtgacagctctaatttctctcgcttggttacctcaagtttttccatgagttctgttgtatccttttcaacaacctcacccatttccaatgtttctgctacaaaagttttgtcttcatcaaagacagaacttttcattttcactgtagttggatttattctttgcaaatgaagctcttcattaagtgctttaagtttacttttatactctaattcctgtttatttttactgtcttctaaatcatcttttactttgagaaggcaagcatactcctcttgtaactcttgatagttaacttcaaagtttttttcagcaaatgaaaaagtgttcctttgcttttcaatctcttcatttagctgaatacattgttgtttgaggtcctcattttcctctataagtatttctatttctttttcccacacagagtctttggatttggacttaatggagtctaagaaaatcaatctttcttcttggctaacaggagtatgtattttcaacatgtcttcaagggttttcttttcatctttaagaatgctattctctgcttcaagttgtgcaaatttttcttgaagatcattctctttttccttcatctgtttttctaacaattctgttttaagttgtaattcttgaacttcttgttcaagtgtacccttttctttttcttcttgtctgagtatttcaatttctttttgaagttcattgatttgaagagtcatttcttctgactttgaatttacaagagactgctgtaaatcttttagctttgaaatttccaaaattaattgattctgcttagttatcaaattgtccttttcaaactgcatggtttctatcttttgactcatttcattctgtaaaccatctatctgctgtttatagtgaatgcctaaattatctttaagtttttcaatatttattcgatgttcaatttctaaatcttccttcagtttggaaagctcttcttcgtgactaaatagaagctgtgttctcagcctctctaattcagcttcttgtgattcagccattctgtctaacacagcattcttttctttttctaacatttcaagttttatcttgtaatttgtaacttctgcttcatgttttaattctagttcctttctggattcagatgcagaaacaatctcagctttcaaatcttccactgtactaagggacttatgtgcttcattaagtttactttcttgttcagctattgtctgtctagctctctgaatctgttcccttgaaaagctcaattcttcaacaaggtcttcaagctgtctctgtagagcacacttttcttctaaaattagtcctagttcttccttgagtttttccttttgagagttagtatcttgcaattttatattcagttcatttattgccacattcattaactttatctgatcttcattaactgtaatatttgaatatgaccttaaagcattctccatttctcccttatgccgtgttttcatttcctccatctgtgccatgtgttgtcttattaattcttgtttcatttgcactatctgctgcccatacatctcatccagctctgcccggagttgttctaactttctttgtgtttcttgttccattcgttgtactatatcagtttcgaactggctgtctttatgatttctcttctgaagttcttcgactgtccccattaactgttttatttcttcagaagactgtctttctttttgcttagaattagtcagctctaatttcatgttttttatttcttggttcttttgcacaatctgttcttgtaattctcctagtaatttatcagcagttgttaatttatcctttagctcaagagttttcttttcttcttctattatttttgtgtttaattcttcaatgattgtctccttttcctgtatttcttctttatttgagttttctacttttttatcttgttccatttcatatactttaattttctcttgcaagaaactaatttgcattgtgaagtcttctttctttttctgataatcttctaataagtggtcttgttcttcaagctgctgttgatgagtgaggatctgttgtttggcttgtagtaagtctgcagctgtgctactatgagtgctgtttctcagagtttcactagcctgtaattgctgaaattgaatctgtaatttttgactctgttctgtcaactctaaaaattctctcattgtctcatccttttctcttcttgcttgttgtaaattagcagtgagctgggttataatgccatctctttgtttaatggcagcttcaaattcttgtaactgctgcagtccttcagtcccataggtaaccctcatttcttccagctctctgtttagctcttcaatctcatgctgcttcccagccaactcactttccatcatctctagatgagtcggactgtcttgtgctccttgttcagaataagaatcatcaacaccaaattcttcttcccttaataaatttgtaggctttcctgttctcatcacaaaactgcaaccatttacctctgaactgcagtcatctgctgtggttgaaatttcactttccagagagttcagtactatctgtggtttcaggtctccactgggggtgttggactatactcttgatatggtttggctgagttcccccatccaaatctcatcttgaattgtagctcccataattcccatgtgtt

SEQ ID NO: 14218 - RNA, 13111 nt, Homo sapiens
  source 1..13111: mol_type = other RNA
gctgggattacaggcatgagccaccgcgcccagcccatatacttaagctgacttttaagagattttgaatatatatgtaaaaatcaccatgactggctctatggcaaggtaggtgagactaatatttagagtttttttaaagtgctctcaaagttggatgttctatacctcatacatttttgaaaaatcttttggtcttcaaaatctgggtcttgtgaaatttggatgctcaaaacaaaacaagcctaggcaaaccaacaaactcagctatgataataaaagtttcctattactacaagatgcttgggtgtaaacaaatgatttcttgaaggaagagataaactactcaatgattcaaagtctctgaatcaggagtgaactgaagtgagatagggaaaagaggttttccttccatgaacagggaatccacctttattttaaagtatgacttgttttttgtttttgaacaaagaaaaaataatccttacaaagtattttaaatgggatagtttttttcgatgatacataaaagcacaatatagtagcagggataatggttacattaagtgcttaaagtaagtgcttcctccttaactccacccgatttgcatgccttaccactttcttttttttttttttttctttgagacagggtctcgctctgctgcccaggctggagtgctgcggcacggccttaccactttctgccatgcgctacttaggaatacgttctccagttaggctctgtagactcagagtaccttgcacactggtgctcattgtgcattttgtgtcatcagtccgctgaatgaacatagtaggaaatcatttttgggaggagtgggatctggggtgataaatcatattttcacttaaattatttaaagtcagtttctctgctggttacaagagtttaagctttggctaacttaataattagctcatgcactaaactggaagctttgattatcctaatgagtgtgaaagaatttcaaagaaaggggagctgtgggtctcgcactgtggtgctgccaagatgtggttaaactcagagcacctgactgtatagttccaagtcgtctttgcagtgcctctagccgagtgatataatctgttagggctctgtcaggatcgtaattctgaagctgagaacatgctaaagaaccaggattgaaatcagctggagtgcctgggtacctattctgaaatggtaaaggggacctaatatagtccagatctgatcttgagcgatacgtagtatgtcttggttctccatataactccagcccaccagaagaatgataaaatgagtcagtcttttctgcaccttgattcagtccaaagccatctctgttaatattgatggaaacagaacctgtgactcgatgccaccgtcgaaccaaaaatttcattctggaaattgcaatggatactctgacggccgaccgaaacctggtgaagccctttgggcgattggtgatcacctctagatccgtgaaagctggctgcccccccatccgggcaagcagggccaaggtggcatcttcacattcctggaacccacccagtaacagcagcaggtatttcttctggtaaatgagagcctttcgaaaactttctgccctcaagtatttaccataaattctctttaaagtgacatgttcagaatcagggctcagagtttgaagtaaagagtcatttcttagttcagctttcagtttgtatacttcagcctctgcccttttcaaagatttctggagagtcaatttttctctgttccatacttctttttcagaggcaatgatggcttcaatgttggcaccaccattcaatgaaaacctggaagaattatctctaccagctcctgtctgtcgataccacctgatctgctcttccagcttcataaccatgttccttaagtcattcttctcttcagtcagttgactgatatgccctgtcagctcagcattttgtctcagtagtctttcagtcaatgagccacaagaagtacttggggacaccaagctgggctcttcaccttgctggccagttaatttctgtagttgtaaaataatttcatcaatattttcctgaacccaaatgaaatcttcatcatctgctgtttcaaactgtagtctctcagaggctttctggggtagaacctgtagttttgaagctacacattgaagcttttgtctgatcatttctaattcatgattacagccggttcctcctccattcatttcaatcaatttagcgtagtttgattcttttgtttctccttctattttctgttgaagaacccaatttctagttctatcactggttaagctccacgtggttggctcattaaggttctgatacagaattcttctactttctcgtttttcttctcgttctagttcttgcttctggaattcctgcatgattccttgtagtcgctgtccttcaaggtctaacttataaacttgttgtcttttctcttccagctggcgctgaagatcttccactttggactggagctcatgcatttttttctgtccctcagtgttggcctcctgttctgtctgcagtgttttcctgtgaacctgcctatctttttccatttgctgtcgtgtttgcaaagaatccagtttatatttttcagtctcatttaacaattctactatgcgactgtgtttttcctctagctgtttctgcagctctttcagtaggtcctctgagggcaagggtggccgagactgtccagtaccatcactgctctgcagctgtgcgtgcaattcccgctccctatctagggtactactcatttcccgaattcgaactttctcagattcaagaagtacctgaagctctaagtttcgaccttgttcttctgacaactgggcatcatatagcattctctgtgattctattttttgctgggattcgttcagtagttgtttctgttgttccaaaagtagatttagctgaagattcctttgtttctgactctcaagtgaaaacttcagatcctcaagttcttctttatcccgttcttcactgcgtcccaacttggctttctctttctccaaagcccactggagctctcttgattttttctgttcacttgctaatgtgtcattaagcaaatgtacttcatctgtcttatctttaacttccaacctgaaagcctccaattcttttaggtgtttatgctgtgccttgagtgttgtttctagttccaatttagtttgtgcaagctcactcttcagttcagcaaccaccattttctcagaactcagctgctcctgcagttccgttgctctgtctttcatactgctgagctccacttgcatctccagcatttgagactgcttctgctgtatattatattccaagagttcttggcttggtttctcactctcttgttctcttttcagagtaattttcctaccattcatttgtgcatgcagtgcctgaatttcagataacaaactccttctatctgctttctggaggcattccatagctgcttgatattcaacaccctgttcttgtattctctgttccaaacagtttagtaaaccaactgcatctgtagtacctagagctgtcagctccgtccgaaatgctgctagtaaaacactacgctcttctaagaaaacttgttgaagggcaagcagtagttcacctcgccagtctgagaagctctcatgagattgagaactatcataaacctcggcttctctttgcagttgcatctttgtaattaaatcctttagagatgagattgtattgatgtaagcttttctctcttctagccaaggttctgaaacctgctgaatagaatggtcctctccatcactatagggagactcagtgagagaaagcacctgcatgccttcattatggacagctctcagtaatccctttattttctttggaaaggaatctgttgcactttcactttcttctcctcggccttctgatgctatgtcaaatccctgactgtgtgtaagataaattccctgaccccagtctgatccagaatcactggagcatatttctctagtctggtaagcatcagaatgtgctagctcaggaattgaggatccctctttacttctcagacactgtatcactgccttcaaggtaccacattcctctttcagtaactgaacggcaacatagtgttccctctttaaggtttcagtttctgaaatatgtctggattccatgtccaaaatttcagcagcatgtagttcttgcatcttctcaattttttcagtaaactgactgattatttcagtaacttcttctgaggaacattcactctgtaaattaatttgtattcctgcatttttaacaagaatttgtggagtctgattgctgctactgatcttcagagtcccatctgtctgggatgcaatgctcttactcagttttataggaagtggctcaaacatgcaggcctttttgctttcttgtacctcagtctcatcttctttttctaaaatggacaatttctcttttgcctctgcgaggtgatccctaacttggcttaagtctttctgaagagatgtcatatttgtttcttttaccaaaagctcttcttgaagtttttcagccttttctttataactggcaagttctgctttggtagccactgattcagctctaagagcctcgagttcattaaaaaatccactttcttcattgctatgaaatagctcagtagttgtcttgagaacttcaacatcttgagggcttcttttcttttctttctctctctgttttttctcattgccctccaatagcttctgtagttctagcagcttcttttctttttctaaaacatttttttctgcaatttctacttgttctttttctaaaatcaaactagtatgcatttcaacaacctggctttctaattctgatattctcaaggttaatgctgatatatctgaccccaactcatcttctcttagttgatttaaattctgaatatttgttctttcaggttctgatgaaattgtttgattatcttgacagaattttgcatattcctgaactgcctcaagttggatttgactgacaagagcagcagccactttttcttcaactattttctgtaggtttacaatcttcttttgaagcatttctgtttcaaactggccttgttcttgcatgtcttttatttgtttataacactgggtaagttctaagtcctttgcactaacagtgctctcaagttgtagcaaccttgtttccaaattaattatggaacctttgccattttcttcaaaagatttgaagtatgtctgattttctagggatttaagagcatcctctgtaaggactacttctagttcaggtttgtctttgctcagatgatctatagccacgttaacactattctctggtatgctttgaatcttttccacactttcacgttctctctttaagctgaataattcctgtgttagctgattcattttaaaattggtttctttaagtacatttttcatgaaggtcatttcttcattagcggtttctacttgctgttccaaggccagcttttcagctataaccacatccaattgatgttttaaactgtctgcttcttctgagagggaatgagcattcattgatgtcttctgtccaatatttgccaattcctgttgaagtttttcaatcacttcattgagctgctctatttcttcttctctatttctcttcacacattcttgatcactcatcaaacattctatttgggtttcaagatcccttatcagttcatttttttcttcaataaccttgttatctgttgtaattttaagttgctgctggagtttcgtaacttgttcatttaattggtcaatttctacctctttttcctgtattatttgagcaaatttcccaaatagcacatgttggtcttgagtagacatggcatcagattcctttatggcaagtcccagtttctccatgtcatccttaaataatttgttttcctgttcaagttcttgtaggcgggtagtagattcctttttctgtatttctaattgcatatgtaattgttgaacttcttcattcttattttccagttcttctctaaactgttctaattgctcttctaagtttgtaatctctttttcctttctgtctatggcatctcgttcagcctgcaattgtacttctagggacaattctggtttagcttctacagctccaaagtgttttcggtcctctaccttttgaaaagtatctgcactcacaagaagcgcctgctccagttctcttactctgaactccagtttctctatttcttcattcctttcttgtatatccctttgaagctgctctttagagagcaaaagctcactgcatttgtctgttttttctttcagatgatttgctaactgttcaacctctctagtttgatgttcactgataggctggaatcgaggaacaaccttaagttgctgttctagtttctgtatttcctgttggaatacatctctctcatgttctctgtcaatggcttgctcatctaaaaattttctcattttttctaactgcttttccaatgcttggttttgctgtcttaaatccattagttcagtatttttttcttgttccagctctataaacctactgacttgttcttccacatctatttctagagctttcacttgtttttgaaggtcatcacgtactttttcagcttgacattgtacttctagtttttccttcattaatttttctgtctcctgtagtaattctgctcctggtgctgcatcgactgcagcatctactagtcgttgttcaactgggcctgcctctgctttcatagcttccttttgtctggacagtaattctctttcttcttggatctgctgttgctctgcctccaattcttgcaacctgttacttgcacataacaactcctgctcaagacgatctattatatcagttttttcctgaatttgcctttcaaaaagagttttttcatctgcatagccatcaatgacgccctcagccttactgagctccacagctagctgttctctggccctggactcctcatgaaggcgctctcgaagttcctcttggcacttaagggactctgttgcttcttgtttctgtctaaatgactcacgcatcaactctgtctgtgtcactttcgcatgttcaagctgactgctagtttcacttatggcttctaggagtttttcaactgctgcttgtagtcgagagctaatgttcagcataagttcttcattttcagggtctatttcagttccagcaaaaccactcctcacaagtcgttgtgacagctctgttccttcctcagttacttttgaccacatgttaatgtcatttcttggcatatcacttccagaataagagggaatggattcatctgtaactcttgtatgttcctcatggacacatgactttacagatgcctctgcttctgacctccaaattaggctggcagatgactggcttttactagatctatctagaatcccaaggacatggcgaccaattgtttcttcaacagctgctgttgtctttacaacttctaagaggatcttcaaaagtctattattagctttctggagtgcatacactgtctttcttgtttgagttccatactgactgcgttccatactgatgatccaatggggaagccaaaatcttaggggccaaattcctccatgcaagctttcattagacaaaatctcaggaggcacatcttcaggttttctgtctaattccttttctttaaatgtttgttcttcaacttctccttggttttcatttccattctgtgtttgcgtactgctgttgcgcagctcacaacacagcttctctcttccagctaaagacagctgctttagtgcttccagctcctctaaaagcaccctctctctctctgaaaccaggttttcattatctatggaggatctctgggctaattgtctattaagtctcttaatctcttcttgtagctgttcctggtcttctcgctgtctctccatttgccgcatatgtgcttgccttaacaattccgttgcctgttgatgttcttggtattgtcgtacaagttcctgtctcatatcttccaactgttcttcattcaacattagttgtctagaagcatccatgcttgacactgaaatctcatcatgaatagactgtctaactataaatgttttatctttggagaacatttcttctgaaatagtcagcacacagtcctttgattctggtatatcatggggatcactatttgataataaaatttcctttccatgttctcctaactctttactaagtggtttaaattcttctttaaatttcacatccactgtctcaaaagtctgaaaaccaatttgatcctgtgataatttcatttcattaaaataatgttgttcttgctgacacacagcatgtgcttgctttgatgatgcagtattttcttttcccccagatattctagacagttcagtttgttgagcaaatgctatactcattgacacaataaccttagctacttcttcttctaattgttcttggtattgtttttcaagcaacttaacgatatttgtttcctctttcactccaaattcaccagaaaactctattgtaccatcaatattctttttcacacaacttccagggtacattgttctctgtgcatcagattctgtaattaccaccgaatcaacaggtaagcttggcggaaccgtggactcactaacagcttgaagcctcttctgtaaacagtggatctctgcctcatagttttgttcagtttctttcaactgttgctgcaaagaggatatgaggctttctaattcttgaacttgttcttcaagtttagttttttcaagatcttgcagagaagataacttgcttttatgattgacatcaatgtcttccaaattggtcatctgagaatggattgataaaaactctgtttcctcttttggaaggttttcttctccaaattcaagtttcataccatctgtctgctgtccccagatcttgcttagtcgtgtttgaagtaccaagagtttgttgtattcttctgttactttgttgagaagagtgtgcatattttcttgaaagtcttgaacttcatatctataatcttgtaattctggatcttcattttcagaaatgtaatcaccagaattctctttgtcttctgcatttacttcacattttaaagcaggagtataatattcaccaaggacactgcataaagtctgtaaaaaataagaacattcttcagacactgccttttgaagttttccaatgagcagatgtaaaggctttccttcatcacctgtttcttgtgttttcatagtctgtagttctaactggtgtattttctgaagttccttgatcttttcctcttgagcaaaaataagctcttctttaagactgcaaagagctttatctttttcattttccatatattcacgaacctgatccacatgagttgaataaaccagagagaggcaaatgcgttgggcttccatctgtagccttaaatcattctgttctgatttaagtacattgagttctttctgaagtttatcattttcacttggttgagttgctctaagtgatgattcctttgttacagatggtaagtgatccaaaatcaactgttcttgcttactttcttctccaacagtcatattttcaaaagaaactttatcttccaccattatttttgattcttcaccaaaacttttatttactttagaaactgatccttcagcacccctgcttgtcatggtcacaactccatctaataaagagcttacttgagtatcacatgactgtacattttctgccctgttgtggttaataatgatttctagctctctacatctcaatgaaacttgttctttctcttgctttaaagatttaacttcttcatttagaaaactaatctcaccatgtttctgtttcaattgttcagaaagatcagacagtctctgtgacagctctaatttctctcgcttggttacctcaagtttttccatgagttctgttgtatccttttcaacaacctcacccatttccaatgtttctgctacaaaagttttgtcttcatcaaagacagaacttttcattttcactgtagttggatttattctttgcaaatgaagctcttcattaagtgctttaagtttacttttatactctaattcctgtttatttttactgtcttctaaatcatcttttactttgagaaggcaagcatactcctcttgtaactcttgatagttaacttcaaagtttttttcagcaaatgaaaaagtgttcctttgcttttcaatctcttcatttagctgaatacattgttgtttgaggtcctcattttcctctataagtatttctatttctttttcccacacagagtctttggatttggacttaatggagtctaagaaaatcaatctttcttcttggctaacaggagtatgtattttcaacatgtcttcaagggttttcttttcatctttaagaatgctattctctgcttcaagttgtgcaaatttttcttgaagatcattctctttttccttcatctgtttttctaacaattctgttttaagttgtaattcttgaacttcttgttcaagtgtacccttttctttttcttcttgtctgagtatttcaatttctttttgaagttcattgatttgaagagtcatttcttctgactttgaatttacaagagactgctgtaaatcttttagctttgaaatttccaaaattaattgattctgcttagttatcaaattgtccttttcaaactgcatggtttctatcttttgactcatttcattctgtaaaccatctatctgctgtttatagtgaatgcctaaattatctttaagtttttcaatatttattcgatgttcaatttctaaatcttccttcagtttggaaagctcttcttcgtgactaaatagaagctgtgttctcagcctctctaattcagcttcttgtgattcagccattctgtctaacacagcattcttttctttttctaacatttcaagttttatcttgtaatttgtaacttctgcttcatgttttaattctagttcctttctggattcagatgcagaaacaatctcagctttcaaatcttccactgtactaagggacttatgtgcttcattaagtttactttcttgttcagctattgtctgtctagctctctgaatctgttcccttgaaaagctcaattcttcaacaaggtcttcaagctgtctctgtagagcacacttttcttctaaaattagtcctagttcttccttgagtttttccttttgagagttagtatcttgcaattttatattcagttcatttattgccacattcattaactttatctgatcttcattaactgtaatatttgaatatgaccttaaagcattctccatttctcccttatgccgtgttttcatttcctccatctgtgccatgtgttgtcttattaattcttgtttcatttgcactatctgctgcccatacatctcatccagctctgcccggagttgttctaactttctttgtgtttcttgttccattcgttgtactatatcagtttcgaactggctgtctttatgatttctcttctgaagttcttcgactgtccccattaactgttttatttcttcagaagactgtctttctttttgcttagaattagtcagctctaatttcatgttttttatttcttggttcttttgcacaatctgttcttgtaattctcctagtaatttatcagcagttgttaatttatcctttagctcaagagttttcttttcttcttctattatttttgtgtttaattcttcaatgattgtctccttttcctgtatttcttctttatttgagttttctacttttttatcttgttccatttcatatactttaattttctcttgcaagaaactaatttgcattgtgaagtcttctttctttttctgataatcttctaataagtggtcttgttcttcaagctgctgttgatgagtgaggatctgttgtttggcttgtagtaagtctgcagctgtgctactatgagtgctgtttctcagagtttcactagcctgtaattgctgaaattgaatctgtaatttttgactctgttctgtcaactctaaaaattctctcattgtctcatccttttctcttcttgcttgttgtaaattagcagtgagctgggttataatgccatctctttgtttaatggcagcttcaaattcttgtaactgctgcagtccttcagtcccataggtaaccctcatttcttccagctctctgtttagctcttcaatctcatgctgcttcccagccaactcactttccatcatctctagatgagtcggactgtcttgtgctccttgttcagaataagaatcatcaacaccaaattcttcttcccttaataaatttgtaggctttcctgttctcatcacaaaactgcaaccatttacctctgaactgcagtcatctgctgtggttgaaatttcactttccagttccacagagaagccctgctcatgactggttatttctccactatgtagagttctcattattgtagattcaggaatcacagttgattctactctctgagaactatttatgtacatttcattacactgtgattgatcaatattcaaatcatggtgtgctgacacatcatgtttactgcttgacgtttttctcttttttttctgcttcttggaaggactctgcccatccgactgagcttttctttgtcgaaactgggcaagcttggctttgccggcctccagcttcttctgtctctcctcgtcctccatggcctctgcaaggaaggcaggggaaaacaggggttgaggggtggttggggatagaaaggaaaggtcgatttggacggaggtgggacggcaagctccacggcctagagagccgattcggtccggcgctcccccgcccgaagtggaagcagtctccgcgctcactggcggatcgtcctcagccgcacgggaagcgccgtcaccgccgccgccgccgccatcttcgtctccacgta

SEQ ID NO: 14219 - RNA, 12770 nt, Homo sapiens
  source 1..12770: mol_type = other RNA
gctgggattacaggcatgagccaccgcgcccagcccatatacttaagctgacttttaagagattttgaatatatatgtaaaaatcaccatgactggctctatggcaaggtaggtgagactaatatttagagtttttttaaagtgctctcaaagttggatgttctatacctcatacatttttgaaaaatcttttggtcttcaaaatctgggtcttgtgaaatttggatgctcaaaacaaaacaagcctaggcaaaccaacaaactcagctatgataataaaagtttcctattactacaagatgcttgggtgtaaacaaatgatttcttgaaggaagagataaactactcaatgattcaaagtctctgaatcaggagtgaactgaagtgagatagggaaaagaggttttccttccatgaacagggaatccacctttattttaaagtatgacttgttttttgtttttgaacaaagaaaaaataatccttacaaagtattttaaatgggatagtttttttcgatgatacataaaagcacaatatagtagcagggataatggttacattaagtgcttaaagtaagtgcttcctccttaactccacccgatttgcatgccttaccactttcttttttttttttttttctttgagacagggtctcgctctgctgcccaggctggagtgctgcggcacggccttaccactttctgccatgcgctacttaggaatacgttctccagttaggctctgtagactcagagtaccttgcacactggtgctcattgtgcattttgtgtcatcagtccgctgaatgaacatagtaggaaatcatttttgggaggagtgggatctggggtgataaatcatattttcacttaaattatttaaagtcagtttctctgctggttacaagagtttaagctttggctaacttaataattagctcatgcactaaactggaagctttgattatcctaatgagtgtgaaagaatttcaaagaaaggggagctgtgggtctcgcactgtggtgctgccaagatgtggttaaactcagagcacctgactgtatagttccaagtcgtctttgcagtgcctctagccgagtgatataatctgttagggctctgtcaggatcgtaattctgaagctgagaacatgctaaagaaccaggattgaaatcagctggagtgcctgggtacctattctgaaatggtaaaggggacctaatatagtccagatctgatcttgagcgatacgtagtatgtcttggttctccatataactccagcccaccagaagaatgataaaatgagtcagtcttttctgcaccttgattcagtccaaagccatctctgttaatattgatggaaacagaacctgtgactcgatgccaccgtcgaaccaaaaatttcattctggaaattgcaatggatactctgacggccgaccgaaacctggtgaagccctttgggcgattggtgatcacctctagatccgtgaaagctggctgcccccccatccgggcaagcagggccaaggtggcatcttcacattcctggaacccacccagtaacagcagcaggtatttcttctggtaaatgagagcctttcgaaaactttctgccctcaagtatttaccataaattctctttaaagtgacatgttcagaatcagggctcagagtttgaagtaaagagtcatttcttagttcagctttcagtttgtatacttcagcctctgcccttttcaaagatttctggagagtcaatttttctctgttccatacttctttttcagaggcaatgatggcttcaatgttggcaccaccattcaatgaaaacctggaagaattatctctaccagctcctgtctgtcgataccacctgatctgctcttccagcttcataaccatgttccttaagtcattcttctcttcagtcagttgactgatatgccctgtcagctcagcattttgtctcagtagtctttcagtcaatgagccacaagaagtacttggggacaccaagctgggctcttcaccttgctggccagttaatttctgtagttgtaaaataatttcatcaatattttcctgaacccaaatgaaatcttcatcatctgctgtttcaaactgtagtctctcagaggctttctggggtagaacctgtagttttgaagctacacattgaagcttttgtctgatcatttctaattcatgattacagccggttcctcctccattcatttcaatcaatttagcgtagtttgattcttttgtttctccttctattttctgttgaagaacccaatttctagttctatcactggttaagctccacgtggttggctcattaaggttctgatacagaattcttctactttctcgtttttcttctcgttctagttcttgcttctggaattcctgcatgattccttgtagtcgctgtccttcaaggtctaacttataaacttgttgtcttttctcttccagctggcgctgaagatcttccactttggactggagctcatgcatttttttctgtccctcagtgttggcctcctgttctgtctgcagtgttttcctgtgaacctgcctatctttttccatttgctgtcgtgtttgcaaagaatccagtttatatttttcagtctcatttaacaattctactatgcgactgtgtttttcctctagctgtttctgcagctctttcagtaggtcctctgagggcaagggtggccgagactgtccagtaccatcactgctctgcagctgtgcgtgcaattcccgctccctatctagggtactactcatttcccgaattcgaactttctcagattcaagaagtacctgaagctctaagtttcgaccttgttcttctgacaactgggcatcatatagcattctctgtgattctattttttgctgggattcgttcagtagttgtttctgttgttccaaaagtagatttagctgaagattcctttgtttctgactctcaagtgaaaacttcagatcctcaagttcttctttatcccgttcttcactgcgtcccaacttggctttctctttctccaaagcccactggagctctcttgattttttctgttcacttgctaatgtgtcattaagcaaatgtacttcatctgtcttatctttaacttccaacctgaaagcctccaattcttttaggtgtttatgctgtgccttgagtgttgtttctagttccaatttagtttgtgcaagctcactcttcagttcagcaaccaccattttctcagaactcagctgctcctgcagttccgttgctctgtctttcatactgctgagctccacttgcatctccagcatttgagactgcttctgctgtatattatattccaagagttcttggcttggtttctcactctcttgttctcttttcagagtaattttcctaccattcatttgtgcatgcagtgcctgaatttcagataacaaactccttctatctgctttctggaggcattccatagctgcttgatattcaacaccctgttcttgtattctctgttccaaacagtttagtaaaccaactgcatctgtagtacctagagctgtcagctccgtccgaaatgctgctagtaaaacactacgctcttctaagaaaacttgttgaagggcaagcagtagttcacctcgccagtctgagaagctctcatgagattgagaactatcataaacctcggcttctctttgcagttgcatctttgtaattaaatcctttagagatgagattgtattgatgtaagcttttctctcttctagccaaggttctgaaacctgctgaatagaatggtcctctccatcactatagggagactcagtgagagaaagcacctgcatgccttcattatggacagctctcagtaatccctttattttctttggaaaggaatctgttgcactttcactttcttctcctcggccttctgatgctatgtcaaatccctgactgtgtgtaagataaattccctgaccccagtctgatccagaatcactggagcatatttctctagtctggtaagcatcagaatgtgctagctcaggaattgaggatccctctttacttctcagacactgtatcactgccttcaaggtaccacattcctctttcagtaactgaacggcaacatagtgttccctctttaaggtttcagtttctgaaatatgtctggattccatgtccaaaatttcagcagcatgtagttcttgcatcttctcaattttttcagtaaactgactgattatttcagtaacttcttctgaggaacattcactctgtaaattaatttgtattcctgcatttttaacaagaatttgtggagtctgattgctgctactgatcttcagagtcccatctgtctgggatgcaatgctcttactcagttttataggaagtggctcaaacatgcaggcctttttgctttcttgtacctcagtctcatcttctttttctaaaatggacaatttctcttttgcctctgcgaggtgatccctaacttggcttaagtctttctgaagagatgtcatatttgtttcttttaccaaaagctcttcttgaagtttttcagccttttctttataactggcaagttctgctttggtagccactgattcagctctaagagcctcgagttcattaaaaaatccactttcttcattgctatgaaatagctcagtagttgtcttgagaacttcaacatcttgagggcttcttttcttttctttctctctctgttttttctcattgccctccaatagcttctgtagttctagcagcttcttttctttttctaaaacatttttttctgcaatttctacttgttctttttctaaaatcaaactagtatgcatttcaacaacctggctttctaattctgatattctcaaggttaatgctgatatatctgaccccaactcatcttctcttagttgatttaaattctgaatatttgttctttcaggttctgatgaaattgtttgattatcttgacagaattttgcatattcctgaactgcctcaagttggatttgactgacaagagcagcagccactttttcttcaactattttctgtaggtttacaatcttcttttgaagcatttctgtttcaaactggccttgttcttgcatgtcttttatttgtttataacactgggtaagttctaagtcctttgcactaacagtgctctcaagttgtagcaaccttgtttccaaattaattatggaacctttgccattttcttcaaaagatttgaagtatgtctgattttctagggatttaagagcatcctctgtaaggactacttctagttcaggtttgtctttgctcagatgatctatagccacgttaacactattctctggtatgctttgaatcttttccacactttcacgttctctctttaagctgaataattcctgtgttagctgattcattttaaaattggtttctttaagtacatttttcatgaaggtcatttcttcattagcggtttctacttgctgttccaaggccagcttttcagctataaccacatccaattgatgttttaaactgtctgcttcttctgagagggaatgagcattcattgatgtcttctgtccaatatttgccaattcctgttgaagtttttcaatcacttcattgagctgctctatttcttcttctctatttctcttcacacattcttgatcactcatcaaacattctatttgggtttcaagatcccttatcagttcatttttttcttcaataaccttgttatctgttgtaattttaagttgctgctggagtttcgtaacttgttcatttaattggtcaatttctacctctttttcctgtattatttgagcaaatttcccaaatagcacatgttggtcttgagtagacatggcatcagattcctttatggcaagtcccagtttctccatgtcatccttaaataatttgttttcctgttcaagttcttgtaggcgggtagtagattcctttttctgtatttctaattgcatatgtaattgttgaacttcttcattcttattttccagttcttctctaaactgttctaattgctcttctaagtttgtaatctctttttcctttctgtctatggcatctcgttcagcctgcaattgtacttctagggacaattctggtttagcttctacagctccaaagtgttttcggtcctctaccttttgaaaagtatctgcactcacaagaagcgcctgctccagttctcttactctgaactccagtttctctatttcttcattcctttcttgtatatccctttgaagctgctctttagagagcaaaagctcactgcatttgtctgttttttctttcagatgatttgctaactgttcaacctctctagtttgatgttcactgataggctggaatcgaggaacaaccttaagttgctgttctagtttctgtatttcctgttggaatacatctctctcatgttctctgtcaatggcttgctcatctaaaaattttctcattttttctaactgcttttccaatgcttggttttgctgtcttaaatccattagttcagtatttttttcttgttccagctctataaacctactgacttgttcttccacatctatttctagagctttcacttgtttttgaaggtcatcacgtactttttcagcttgacattgtacttctagtttttccttcattaatttttctgtctcctgtagtaattctgctcctggtgctgcatcgactgcagcatctactagtcgttgttcaactgggcctgcctctgctttcatagcttccttttgtctggacagtaattctctttcttcttggatctgctgttgctctgcctccaattcttgcaacctgttacttgcacataacaactcctgctcaagacgatctattatatcagttttttcctgaatttgcctttcaaaaagagttttttcatctgcatagccatcaatgacgccctcagccttactgagctccacagctagctgttctctggccctggactcctcatgaaggcgctctcgaagttcctcttggcacttaagggactctgttgcttcttgtttctgtctaaatgactcacgcatcaactctgtctgtgtcactttcgcatgttcaagctgactgctagtttcacttatggcttctaggagtttttcaactgctgcttgtagtcgagagctaatgttcagcataagttcttcattttcagggtctatttcagttccagcaaaaccactcctcacaagtcgttgtgacagctctgttccttcctcagttacttttgaccacatgttaatgtcatttcttggcatatcacttccagaataagagggaatggattcatctgtaactcttgtatgttcctcatggacacatgactttacagatgcctctgcttctgacctccaaattaggctggcagatgactggcttttactagatctatctagaatcccaaggacatggcgaccaattgtttcttcaacagctgctgttgtctttacaacttctaagaggatcttcaaaagtctattattagctttctggagtgcatacactgtctttcttgtttgagttccatactgactgcgttccatactgatgatccaatggggaagccaaaatcttaggggccaaattcctccatgcaagctttcattagacaaaatctcaggaggcacatcttcaggttttctgtctaattccttttctttaaatgtttgttcttcaacttctccttggttttcatttccattctgtgtttgcgtactgctgttgcgcagctcacaacacagcttctctcttccagctaaagacagctgctttagtgcttccagctcctctaaaagcaccctctctctctctgaaaccaggttttcattatctatggaggatctctgggctaattgtctattaagtctcttaatctcttcttgtagctgttcctggtcttctcgctgtctctccatttgccgcatatgtgcttgccttaacaattccgttgcctgttgatgttcttggtattgtcgtacaagttcctgtctcatatcttccaactgttcttcattcaacattagttgtctagaagcatccatgcttgacactgaaatctcatcatgaatagactgtctaactataaatgttttatctttggagaacatttcttctgaaatagtcagcacacagtcctttgattctggtatatcatggggatcactatttgataataaaatttcctttccatgttctcctaactctttactaagtggtttaaattcttctttaaatttcacatccactgtctcaaaagtctgaaaaccaatttgatcctgtgataatttcatttcattaaaataatgttgttcttgctgacacacagcatgtgcttgctttgatgatgcagtattttcttttcccccagatattctagacagttcagtttgttgagcaaatgctatactcattgacacaataaccttagctacttcttcttctaattgttcttggtattgtttttcaagcaacttaacgatatttgtttcctctttcactccaaattcaccagaaaactctattgtaccatcaatattctttttcacacaacttccagggtacattgttctctgtgcatcagattctgtaattaccaccgaatcaacaggtaagcttggcggaaccgtggactcactaacagcttgaagcctcttctgtaaacagtggatctctgcctcatagttttgttcagtttctttcaactgttgctgcaaagaggatatgaggctttctaattcttgaacttgttcttcaagtttagttttttcaagatcttgcagagaagataacttgcttttatgattgacatcaatgtcttccaaattggtcatctgagaatggattgataaaaactctgtttcctcttttggaaggttttcttctccaaattcaagtttcataccatctgtctgctgtccccagatcttgcttagtcgtgtttgaagtaccaagagtttgttgtattcttctgttactttgttgagaagagtgtgcatattttcttgaaagtcttgaacttcatatctataatcttgtaattctggatcttcattttcagaaatgtaatcaccagaattctctttgtcttctgcatttacttcacattttaaagcaggagtataatattcaccaaggacactgcataaagtctgtaaaaaataagaacattcttcagacactgccttttgaagttttccaatgagcagatgtaaaggctttccttcatcacctgtttcttgtgttttcatagtctgtagttctaactggtgtattttctgaagttccttgatcttttcctcttgagcaaaaataagctcttctttaagactgcaaagagctttatctttttcattttccatatattcacgaacctgatccacatgagttgaataaaccagagagaggcaaatgcgttgggcttccatctgtagccttaaatcattctgttctgatttaagtacattgagttctttctgaagtttatcattttcacttggttgagttgctctaagtgatgattcctttgttacagatggtaagtgatccaaaatcaactgttcttgcttactttcttctccaacagtcatattttcaaaagaaactttatcttccaccattatttttgattcttcaccaaaacttttatttactttagaaactgatccttcagcacccctgcttgtcatggtcacaactccatctaataaagagcttacttgagtatcacatgactgtacattttctgccctgttgtggttaataatgatttctagctctctacatctcaatgaaacttgttctttctcttgctttaaagatttaacttcttcatttagaaaactaatctcaccatgtttctgtttcaattgttcagaaagatcagacagtctctgtgacagctctaatttctctcgcttggttacctcaagtttttccatgagttctgttgtatccttttcaacaacctcacccatttccaatgtttctgctacaaaagttttgtcttcatcaaagacagaacttttcattttcactgtagttggatttattctttgcaaatgaagctcttcattaagtgctttaagtttacttttatactctaattcctgtttatttttactgtcttctaaatcatcttttactttgagaaggcaagcatactcctcttgtaactcttgatagttaacttcaaagtttttttcagcaaatgaaaaagtgttcctttgcttttcaatctcttcatttagctgaatacattgttgtttgaggtcctcattttcctctataagtatttctatttctttttcccacacagagtctttggatttggacttaatggagtctaagaaaatcaatctttcttcttggctaacaggagtatgtattttcaacatgtcttcaagggttttcttttcatctttaagaatgctattctctgcttcaagttgtgcaaatttttcttgaagatcattctctttttccttcatctgtttttctaacaattctgttttaagttgtaattcttgaacttcttgttcaagtgtacccttttctttttcttcttgtctgagtatttcaatttctttttgaagttcattgatttgaagagtcatttcttctgactttgaatttacaagagactgctgtaaatcttttagctttgaaatttccaaaattaattgattctgcttagttatcaaattgtccttttcaaactgcatggtttctatcttttgactcatttcattctgtaaaccatctatctgctgtttatagtgaatgcctaaattatctttaagtttttcaatatttattcgatgttcaatttctaaatcttccttcagtttggaaagctcttcttcgtgactaaatagaagctgtgttctcagcctctctaattcagcttcttgtgattcagccattctgtctaacacagcattcttttctttttctaacatttcaagttttatcttgtaatttgtaacttctgcttcatgttttaattctagttcctttctggattcagatgcagaaacaatctcagctttcaaatcttccactgtactaagggacttatgtgcttcattaagtttactttcttgttcagctattgtctgtctagctctctgaatctgttcccttgaaaagctcaattcttcaacaaggtcttcaagctgtctctgtagagcacacttttcttctaaaattagtcctagttcttccttgagtttttccttttgagagttagtatcttgcaattttatattcagttcatttattgccacattcattaactttatctgatcttcattaactgtaatatttgaatatgaccttaaagcattctccatttctcccttatgccgtgttttcatttcctccatctgtgccatgtgttgtcttattaattcttgtttcatttgcactatctgctgcccatacatctcatccagctctgcccggagttgttctaactttctttgtgtttcttgttccattcgttgtactatatcagtttcgaactggctgtctttatgatttctcttctgaagttcttcgactgtccccattaactgttttatttcttcagaagactgtctttctttttgcttagaattagtcagctctaatttcatgttttttatttcttggttcttttgcacaatctgttcttgtaattctcctagtaatttatcagcagttgttaatttatcctttagctcaagagttttcttttcttcttctattatttttgtgtttaattcttcaatgattgtctccttttcctgtatttcttctttatttgagttttctacttttttatcttgttccatttcatatactttaattttctcttgcaagaaactaatttgcattgtgaagtcttctttctttttctgataatcttctaataagtggtcttgttcttcaagctgctgttgatgagtgaggatctgttgtttggcttgtagtaagtctgcagctgtgctactatgagtgctgtttctcagagtttcactagcctgtaattgctgaaattgaatctgtaatttttgactctgttctgtcaactctaaaaattctctcattgtctcatccttttctcttcttgcttgttgtaaattagcagtgagctgggttataatgccatctctttgtttaatggcagcttcaaattcttgtaactgctgcagtccttcagtcccataggtaaccctcatttcttccagctctctgtttagctcttcaatctcatgctgcttcccagccaactcactttccatcatctctagatgagtcggactgtcttgtgctccttgttcagaataagaatcatcaacaccaaattcttcttcccttaataaatttgtaggctttcctgttctcatcacaaaactgcaaccatttactgaatacactgagttgctaaaccattcagagtacagaatagtttatagtctcctcaaattctggagtaaagaaatgacaatcacatctctgaactgcagtcatctgctgtggttgaaatttcactttccagttccacagagaagccctgctcatgactggttatttctccactatgtagagttctcattattgtagattcaggaatcacagttgattctactctctgagaactatttatgtac

SEQ ID NO: 14220 - RNA, 13057 nt, Homo sapiens
  source 1..13057: mol_type = other RNA
gctgggattacaggcatgagccaccgcgcccagcccatatacttaagctgacttttaagagattttgaatatatatgtaaaaatcaccatgactggctctatggcaaggtaggtgagactaatatttagagtttttttaaagtgctctcaaagttggatgttctatacctcatacatttttgaaaaatcttttggtcttcaaaatctgggtcttgtgaaatttggatgctcaaaacaaaacaagcctaggcaaaccaacaaactcagctatgataataaaagtttcctattactacaagatgcttgggtgtaaacaaatgatttcttgaaggaagagataaactactcaatgattcaaagtctctgaatcaggagtgaactgaagtgagatagggaaaagaggttttccttccatgaacagggaatccacctttattttaaagtatgacttgttttttgtttttgaacaaagaaaaaataatccttacaaagtattttaaatgggatagtttttttcgatgatacataaaagcacaatatagtagcagggataatggttacattaagtgcttaaagtaagtgcttcctccttaactccacccgatttgcatgccttaccactttcttttttttttttttttctttgagacagggtctcgctctgctgcccaggctggagtgctgcggcacggccttaccactttctgccatgcgctacttaggaatacgttctccagttaggctctgtagactcagagtaccttgcacactggtgctcattgtgcattttgtgtcatcagtccgctgaatgaacatagtaggaaatcatttttgggaggagtgggatctggggtgataaatcatattttcacttaaattatttaaagtcagtttctctgctggttacaagagtttaagctttggctaacttaataattagctcatgcactaaactggaagctttgattatcctaatgagtgtgaaagaatttcaaagaaaggggagctgtgggtctcgcactgtggtgctgccaagatgtggttaaactcagagcacctgactgtatagttccaagtcgtctttgcagtgcctctagccgagtgatataatctgttagggctctgtcaggatcgtaattctgaagctgagaacatgctaaagaaccaggattgaaatcagctggagtgcctgggtacctattctgaaatggtaaaggggacctaatatagtccagatctgatcttgagcgatacgtagtatgtcttggttctccatataactccagcccaccagaagaatgataaaatgagtcagtcttttctgcaccttgattcagtccaaagccatctctgttaatattgatggaaacagaacctgtgactcgatgccaccgtcgaaccaaaaatttcattctggaaattgcaatggatactctgacggccgaccgaaacctggtgaagccctttgggcgattggtgatcacctctagatccgtgaaagctggctgcccccccatccgggcaagcagggccaaggtggcatcttcacattcctggaacccacccagtaacagcagcaggtatttcttctggtaaatgagagcctttcgaaaactttctgccctcaagtatttaccataaattctctttaaagtgacatgttcagaatcagggctcagagtttgaagtaaagagtcatttcttagttcagctttcagtttgtatacttcagcctctgcccttttcaaagatttctggagagtcaatttttctctgttccatacttctttttcagaggcaatgatggcttcaatgttggcaccaccattcaatgaaaacctggaagaattatctctaccagctcctgtctgtcgataccacctgatctgctcttccagcttcataaccatgttccttaagtcattcttctcttcagtcagttgactgatatgccctgtcagctcagcattttgtctcagtagtctttcagtcaatgagccacaagaagtacttggggacaccaagctgggctcttcaccttgctggccagttaatttctgtagttgtaaaataatttcatcaatattttcctgaacccaaatgaaatcttcatcatctgctgtttcaaactgtagtctctcagaggctttctggggtagaacctgtagttttgaagctacacattgaagcttttgtctgatcatttctaattcatgattacagccggttcctcctccattcatttcaatcaatttagcgtagtttgattcttttgtttctccttctattttctgttgaagaacccaatttctagttctatcactggttaagctccacgtggttggctcattaaggttctgatacagaattcttctactttctcgtttttcttctcgttctagttcttgcttctggaattcctgcatgattccttgtagtcgctgtccttcaaggtctaacttataaacttgttgtcttttctcttccagctggcgctgaagatcttccactttggactggagctcatgcatttttttctgtccctcagtgttggcctcctgttctgtctgcagtgttttcctgtgaacctgcctatctttttccatttgctgtcgtgtttgcaaagaatccagtttatatttttcagtctcatttaacaattctactatgcgactgtgtttttcctctagctgtttctgcagctctttcagtaggtcctctgagggcaagggtggccgagactgtccagtaccatcactgctctgcagctgtgcgtgcaattcccgctccctatctagggtactactcatttcccgaattcgaactttctcagattcaagaagtacctgaagctctaagtttcgaccttgttcttctgacaactgggcatcatatagcattctctgtgattctattttttgctgggattcgttcagtagttgtttctgttgttccaaaagtagatttagctgaagattcctttgtttctgactctcaagtgaaaacttcagatcctcaagttcttctttatcccgttcttcactgcgtcccaacttggctttctctttctccaaagcccactggagctctcttgattttttctgttcacttgctaatgtgtcattaagcaaatgtacttcatctgtcttatctttaacttccaacctgaaagcctccaattcttttaggtgtttatgctgtgccttgagtgttgtttctagttccaatttagtttgtgcaagctcactcttcagttcagcaaccaccattttctcagaactcagctgctcctgcagttccgttgctctgtctttcatactgctgagctccacttgcatctccagcatttgagactgcttctgctgtatattatattccaagagttcttggcttggtttctcactctcttgttctcttttcagagtaattttcctaccattcatttgtgcatgcagtgcctgaatttcagataacaaactccttctatctgctttctggaggcattccatagctgcttgatattcaacaccctgttcttgtattctctgttccaaacagtttagtaaaccaactgcatctgtagtacctagagctgtcagctccgtccgaaatgctgctagtaaaacactacgctcttctaagaaaacttgttgaagggcaagcagtagttcacctcgccagtctgagaagctctcatgagattgagaactatcataaacctcggcttctctttgcagttgcatctttgtaattaaatcctttagagatgagattgtattgatgtaagcttttctctcttctagccaaggttctgaaacctgctgaatagaatggtcctctccatcactatagggagactcagtgagagaaagcacctgcatgccttcattatggacagctctcagtaatccctttattttctttggaaaggaatctgttgcactttcactttcttctcctcggccttctgatgctatgtcaaatccctgactgtgtgtaagataaattccctgaccccagtctgatccagaatcactggagcatatttctctagtctggtaagcatcagaatgtgctagctcaggaattgaggatccctctttacttctcagacactgtatcactgccttcaaggtaccacattcctctttcagtaactgaacggcaacatagtgttccctctttaaggtttcagtttctgaaatatgtctggattccatgtccaaaatttcagcagcatgtagttcttgcatcttctcaattttttcagtaaactgactgattatttcagtaacttcttctgaggaacattcactctgtaaattaatttgtattcctgcatttttaacaagaatttgtggagtctgattgctgctactgatcttcagagtcccatctgtctgggatgcaatgctcttactcagttttataggaagtggctcaaacatgcaggcctttttgctttcttgtacctcagtctcatcttctttttctaaaatggacaatttctcttttgcctctgcgaggtgatccctaacttggcttaagtctttctgaagagatgtcatatttgtttcttttaccaaaagctcttcttgaagtttttcagccttttctttataactggcaagttctgctttggtagccactgattcagctctaagagcctcgagttcattaaaaaatccactttcttcattgctatgaaatagctcagtagttgtcttgagaacttcaacatcttgagggcttcttttcttttctttctctctctgttttttctcattgccctccaatagcttctgtagttctagcagcttcttttctttttctaaaacatttttttctgcaatttctacttgttctttttctaaaatcaaactagtatgcatttcaacaacctggctttctaattctgatattctcaaggttaatgctgatatatctgaccccaactcatcttctcttagttgatttaaattctgaatatttgttctttcaggttctgatgaaattgtttgattatcttgacagaattttgcatattcctgaactgcctcaagttggatttgactgacaagagcagcagccactttttcttcaactattttctgtaggtttacaatcttcttttgaagcatttctgtttcaaactggccttgttcttgcatgtcttttatttgtttataacactgggtaagttctaagtcctttgcactaacagtgctctcaagttgtagcaaccttgtttccaaattaattatggaacctttgccattttcttcaaaagatttgaagtatgtctgattttctagggatttaagagcatcctctgtaaggactacttctagttcaggtttgtctttgctcagatgatctatagccacgttaacactattctctggtatgctttgaatcttttccacactttcacgttctctctttaagctgaataattcctgtgttagctgattcattttaaaattggtttctttaagtacatttttcatgaaggtcatttcttcattagcggtttctacttgctgttccaaggccagcttttcagctataaccacatccaattgatgttttaaactgtctgcttcttctgagagggaatgagcattcattgatgtcttctgtccaatatttgccaattcctgttgaagtttttcaatcacttcattgagctgctctatttcttcttctctatttctcttcacacattcttgatcactcatcaaacattctatttgggtttcaagatcccttatcagttcatttttttcttcaataaccttgttatctgttgtaattttaagttgctgctggagtttcgtaacttgttcatttaattggtcaatttctacctctttttcctgtattatttgagcaaatttcccaaatagcacatgttggtcttgagtagacatggcatcagattcctttatggcaagtcccagtttctccatgtcatccttaaataatttgttttcctgttcaagttcttgtaggcgggtagtagattcctttttctgtatttctaattgcatatgtaattgttgaacttcttcattcttattttccagttcttctctaaactgttctaattgctcttctaagtttgtaatctctttttcctttctgtctatggcatctcgttcagcctgcaattgtacttctagggacaattctggtttagcttctacagctccaaagtgttttcggtcctctaccttttgaaaagtatctgcactcacaagaagcgcctgctccagttctcttactctgaactccagtttctctatttcttcattcctttcttgtatatccctttgaagctgctctttagagagcaaaagctcactgcatttgtctgttttttctttcagatgatttgctaactgttcaacctctctagtttgatgttcactgataggctggaatcgaggaacaaccttaagttgctgttctagtttctgtatttcctgttggaatacatctctctcatgttctctgtcaatggcttgctcatctaaaaattttctcattttttctaactgcttttccaatgcttggttttgctgtcttaaatccattagttcagtatttttttcttgttccagctctataaacctactgacttgttcttccacatctatttctagagctttcacttgtttttgaaggtcatcacgtactttttcagcttgacattgtacttctagtttttccttcattaatttttctgtctcctgtagtaattctgctcctggtgctgcatcgactgcagcatctactagtcgttgttcaactgggcctgcctctgctttcatagcttccttttgtctggacagtaattctctttcttcttggatctgctgttgctctgcctccaattcttgcaacctgttacttgcacataacaactcctgctcaagacgatctattatatcagttttttcctgaatttgcctttcaaaaagagttttttcatctgcatagccatcaatgacgccctcagccttactgagctccacagctagctgttctctggccctggactcctcatgaaggcgctctcgaagttcctcttggcacttaagggactctgttgcttcttgtttctgtctaaatgactcacgcatcaactctgtctgtgtcactttcgcatgttcaagctgactgctagtttcacttatggcttctaggagtttttcaactgctgcttgtagtcgagagctaatgttcagcataagttcttcattttcagggtctatttcagttccagcaaaaccactcctcacaagtcgttgtgacagctctgttccttcctcagttacttttgaccacatgttaatgtcatttcttggcatatcacttccagaataagagggaatggattcatctgtaactcttgtatgttcctcatggacacatgactttacagatgcctctgcttctgacctccaaattaggctggcagatgactggcttttactagatctatctagaatcccaaggacatggcgaccaattgtttcttcaacagctgctgttgtctttacaacttctaagaggatcttcaaaagtctattattagctttctggagtgcatacactgtctttcttgtttgagttccatactgactgcgttccatactgatgatccaatggggaagccaaaatcttaggggccaaattcctccatgcaagctttcattagacaaaatctcaggaggcacatcttcaggttttctgtctaattccttttctttaaatgtttgttcttcaacttctccttggttttcatttccattctgtgtttgcgtactgctgttgcgcagctcacaacacagcttctctcttccagctaaagacagctgctttagtgcttccagctcctctaaaagcaccctctctctctctgaaaccaggttttcattatctatggaggatctctgggctaattgtctattaagtctcttaatctcttcttgtagctgttcctggtcttctcgctgtctctccatttgccgcatatgtgcttgccttaacaattccgttgcctgttgatgttcttggtattgtcgtacaagttcctgtctcatatcttccaactgttcttcattcaacattagttgtctagaagcatccatgcttgacactgaaatctcatcatgaatagactgtctaactataaatgttttatctttggagaacatttcttctgaaatagtcagcacacagtcctttgattctggtatatcatggggatcactatttgataataaaatttcctttccatgttctcctaactctttactaagtggtttaaattcttctttaaatttcacatccactgtctcaaaagtctgaaaaccaatttgatcctgtgataatttcatttcattaaaataatgttgttcttgctgacacacagcatgtgcttgctttgatgatgcagtattttcttttcccccagatattctagacagttcagtttgttgagcaaatgctatactcattgacacaataaccttagctacttcttcttctaattgttcttggtattgtttttcaagcaacttaacgatatttgtttcctctttcactccaaattcaccagaaaactctattgtaccatcaatattctttttcacacaacttccagggtacattgttctctgtgcatcagattctgtaattaccaccgaatcaacaggtaagcttggcggaaccgtggactcactaacagcttgaagcctcttctgtaaacagtggatctctgcctcatagttttgttcagtttctttcaactgttgctgcaaagaggatatgaggctttctaattcttgaacttgttcttcaagtttagttttttcaagatcttgcagagaagataacttgcttttatgattgacatcaatgtcttccaaattggtcatctgagaatggattgataaaaactctgtttcctcttttggaaggttttcttctccaaattcaagtttcataccatctgtctgctgtccccagatcttgcttagtcgtgtttgaagtaccaagagtttgttgtattcttctgttactttgttgagaagagtgtgcatattttcttgaaagtcttgaacttcatatctataatcttgtaattctggatcttcattttcagaaatgtaatcaccagaattctctttgtcttctgcatttacttcacattttaaagcaggagtataatattcaccaaggacactgcataaagtctgtaaaaaataagaacattcttcagacactgccttttgaagttttccaatgagcagatgtaaaggctttccttcatcacctgtttcttgtgttttcatagtctgtagttctaactggtgtattttctgaagttccttgatcttttcctcttgagcaaaaataagctcttctttaagactgcaaagagctttatctttttcattttccatatattcacgaacctgatccacatgagttgaataaaccagagagaggcaaatgcgttgggcttccatctgtagccttaaatcattctgttctgatttaagtacattgagttctttctgaagtttatcattttcacttggttgagttgctctaagtgatgattcctttgttacagatggtaagtgatccaaaatcaactgttcttgcttactttcttctccaacagtcatattttcaaaagaaactttatcttccaccattatttttgattcttcaccaaaacttttatttactttagaaactgatccttcagcacccctgcttgtcatggtcacaactccatctaataaagagcttacttgagtatcacatgactgtacattttctgccctgttgtggttaataatgatttctagctctctacatctcaatgaaacttgttctttctcttgctttaaagatttaacttcttcatttagaaaactaatctcaccatgtttctgtttcaattgttcagaaagatcagacagtctctgtgacagctctaatttctctcgcttggttacctcaagtttttccatgagttctgttgtatccttttcaacaacctcacccatttccaatgtttctgctacaaaagttttgtcttcatcaaagacagaacttttcattttcactgtagttggatttattctttgcaaatgaagctcttcattaagtgctttaagtttacttttatactctaattcctgtttatttttactgtcttctaaatcatcttttactttgagaaggcaagcatactcctcttgtaactcttgatagttaacttcaaagtttttttcagcaaatgaaaaagtgttcctttgcttttcaatctcttcatttagctgaatacattgttgtttgaggtcctcattttcctctataagtatttctatttctttttcccacacagagtctttggatttggacttaatggagtctaagaaaatcaatctttcttcttggctaacaggagtatgtattttcaacatgtcttcaagggttttcttttcatctttaagaatgctattctctgcttcaagttgtgcaaatttttcttgaagatcattctctttttccttcatctgtttttctaacaattctgttttaagttgtaattcttgaacttcttgttcaagtgtacccttttctttttcttcttgtctgagtatttcaatttctttttgaagttcattgatttgaagagtcatttcttctgactttgaatttacaagagactgctgtaaatcttttagctttgaaatttccaaaattaattgattctgcttagttatcaaattgtccttttcaaactgcatggtttctatcttttgactcatttcattctgtaaaccatctatctgctgtttatagtgaatgcctaaattatctttaagtttttcaatatttattcgatgttcaatttctaaatcttccttcagtttggaaagctcttcttcgtgactaaatagaagctgtgttctcagcctctctaattcagcttcttgtgattcagccattctgtctaacacagcattcttttctttttctaacatttcaagttttatcttgtaatttgtaacttctgcttcatgttttaattctagttcctttctggattcagatgcagaaacaatctcagctttcaaatcttccactgtactaagggacttatgtgcttcattaagtttactttcttgttcagctattgtctgtctagctctctgaatctgttcccttgaaaagctcaattcttcaacaaggtcttcaagctgtctctgtagagcacacttttcttctaaaattagtcctagttcttccttgagtttttccttttgagagttagtatcttgcaattttatattcagttcatttattgccacattcattaactttatctgatcttcattaactgtaatatttgaatatgaccttaaagcattctccatttctcccttatgccgtgttttcatttcctccatctgtgccatgtgttgtcttattaattcttgtttcatttgcactatctgctgcccatacatctcatccagctctgcccggagttgttctaactttctttgtgtttcttgttccattcgttgtactatatcagtttcgaactggctgtctttatgatttctcttctgaagttcttcgactgtccccattaactgttttatttcttcagaagactgtctttctttttgcttagaattagtcagctctaatttcatgttttttatttcttggttcttttgcacaatctgttcttgtaattctcctagtaatttatcagcagttgttaatttatcctttagctcaagagttttcttttcttcttctattatttttgtgtttaattcttcaatgattgtctccttttcctgtatttcttctttatttgagttttctacttttttatcttgttccatttcatatactttaattttctcttgcaagaaactaatttgcattgtgaagtcttctttctttttctgataatcttctaataagtggtcttgttcttcaagctgctgttgatgagtgaggatctgttgtttggcttgtagtaagtctgcagctgtgctactatgagtgctgtttctcagagtttcactagcctgtaattgctgaaattgaatctgtaatttttgactctgttctgtcaactctaaaaattctctcattgtctcatccttttctcttcttgcttgttgtaaattagcagtgagctgggttataatgccatctctttgtttaatggcagcttcaaattcttgtaactgctgcagtccttcagtcccataggtaaccctcatttcttccagctctctgtttagctcttcaatctcatgctgcttcccagccaactcactttccatcatctctagatgagtcggactgtcttgtgctccttgttcagaataagaatcatcaacaccaaattcttcttcctctgaactgcagtcatctgctgtggttgaaatttcactttccagttccacagagaagccctgctcatgactggttatttctccactatgtagagttctcattattgtagattcaggaatcacagttgattctactctctgagaactatttatgtacatttcattacactgtgattgatcaatattcaaatcatggtgtgctgacacatcatgtttactgcttgacgtttttctcttttttttctgcttcttggaaggactctgcccatccgactgagcttttctttgtcgaaactgggcaagcttggctttgccggcctccagcttcttctgtctctcctcgtcctccatggcctctgcaaggaaggcaggggaaaacaggggttgaggggtggttggggatagaaaggaaaggtcgatttggacggaggtgggacggcaagctccacggcctagagagccgattcggtccggcgctcccccgcccgaagtggaagcagtctccgcgctcactggcggatcgtcctcagccgcacgggaagcgccgtcaccgccgccgccgccgccatcttcgtctccacgta

SEQ ID NO: 14221 - RNA, 12874 nt, Homo sapiens
  source 1..12874: mol_type = other RNA
gctgggattacaggcatgagccaccgcgcccagcccatatacttaagctgacttttaagagattttgaatatatatgtaaaaatcaccatgactggctctatggcaaggtaggtgagactaatatttagagtttttttaaagtgctctcaaagttggatgttctatacctcatacatttttgaaaaatcttttggtcttcaaaatctgggtcttgtgaaatttggatgctcaaaacaaaacaagcctaggcaaaccaacaaactcagctatgataataaaagtttcctattactacaagatgcttgggtgtaaacaaatgatttcttgaaggaagagataaactactcaatgattcaaagtctctgaatcaggagtgaactgaagtgagatagggaaaagaggttttccttccatgaacagggaatccacctttattttaaagtatgacttgttttttgtttttgaacaaagaaaaaataatccttacaaagtattttaaatgggatagtttttttcgatgatacataaaagcacaatatagtagcagggataatggttacattaagtgcttaaagtaagtgcttcctccttaactccacccgatttgcatgccttaccactttcttttttttttttttttctttgagacagggtctcgctctgctgcccaggctggagtgctgcggcacggccttaccactttctgccatgcgctacttaggaatacgttctccagttaggctctgtagactcagagtaccttgcacactggtgctcattgtgcattttgtgtcatcagtccgctgaatgaacatagtaggaaatcatttttgggaggagtgggatctggggtgataaatcatattttcacttaaattatttaaagtcagtttctctgctggttacaagagtttaagctttggctaacttaataattagctcatgcactaaactggaagctttgattatcctaatgagtgtgaaagaatttcaaagaaaggggagctgtgggtctcgcactgtggtgctgccaagatgtggttaaactcagagcacctgactgtatagttccaagtcgtctttgcagtgcctctagccgagtgatataatctgttagggctctgtcaggatcgtaattctgaagctgagaacatgctaaagaaccaggattgaaatcagctggagtgcctgggtacctattctgaaatggtaaaggggacctaatatagtccagatctgatcttgagcgatacgtagtatgtcttggttctccatataactccagcccaccagaagaatgataaaatgagtcagtcttttctgcaccttgattcagtccaaagccatctctgttaatattgatggaaacagaacctgtgactcgatgccaccgtcgaaccaaaaatttcattctggaaattgcaatggatactctgacggccgaccgaaacctggtgaagccctttgggcgattggtgatcacctctagatccgtgaaagctggctgcccccccatccgggcaagcagggccaaggtggcatcttcacattcctggaacccacccagtaacagcagcaggtatttcttctggtaaatgagagcctttcgaaaactttctgccctcaagtatttaccataaattctctttaaagtgacatgttcagaatcagggctcagagtttgaagtaaagagtcatttcttagttcagctttcagtttgtatacttcagcctctgcccttttcaaagatttctggagagtcaatttttctctgttccatacttctttttcagaggcaatgatggcttcaatgttggcaccaccattcaatgaaaacctggaagaattatctctaccagctcctgtctgtcgataccacctgatctgctcttccagcttcataaccatgttccttaagtcattcttctcttcagtcagttgactgatatgccctgtcagctcagcattttgtctcagtagtctttcagtcaatgagccacaagaagtacttggggacaccaagctgggctcttcaccttgctggccagttaatttctgtagttgtaaaataatttcatcaatattttcctgaacccaaatgaaatcttcatcatctgctgtttcaaactgtagtctctcagaggctttctggggtagaacctgtagttttgaagctacacattgaagcttttgtctgatcatttctaattcatgattacagccggttcctcctccattcatttcaatcaatttagcgtagtttgattcttttgtttctccttctattttctgttgaagaacccaatttctagttctatcactggttaagctccacgtggttggctcattaaggttctgatacagaattcttctactttctcgtttttcttctcgttctagttcttgcttctggaattcctgcatgattccttgtagtcgctgtccttcaaggtctaacttataaacttgttgtcttttctcttccagctggcgctgaagatcttccactttggactggagctcatgcatttttttctgtccctcagtgttggcctcctgttctgtctgcagtgttttcctgtgaacctgcctatctttttccatttgctgtcgtgtttgcaaagaatccagtttatatttttcagtctcatttaacaattctactatgcgactgtgtttttcctctagctgtttctgcagctctttcagtaggtcctctgagggcaagggtggccgagactgtccagtaccatcactgctctgcagctgtgcgtgcaattcccgctccctatctagggtactactcatttcccgaattcgaactttctcagattcaagaagtacctgaagctctaagtttcgaccttgttcttctgacaactgggcatcatatagcattctctgtgattctattttttgctgggattcgttcagtagttgtttctgttgttccaaaagtagatttagctgaagattcctttgtttctgactctcaagtgaaaacttcagatcctcaagttcttctttatcccgttcttcactgcgtcccaacttggctttctctttctccaaagcccactggagctctcttgattttttctgttcacttgctaatgtgtcattaagcaaatgtacttcatctgtcttatctttaacttccaacctgaaagcctccaattcttttaggtgtttatgctgtgccttgagtgttgtttctagttccaatttagtttgtgcaagctcactcttcagttcagcaaccaccattttctcagaactcagctgctcctgcagttccgttgctctgtctttcatactgctgagctccacttgcatctccagcatttgagactgcttctgctgtatattatattccaagagttcttggcttggtttctcactctcttgttctcttttcagagtaattttcctaccattcatttgtgcatgcagtgcctgaatttcagataacaaactccttctatctgctttctggaggcattccatagctgcttgatattcaacaccctgttcttgtattctctgttccaaacagtttagtaaaccaactgcatctgtagtacctagagctgtcagctccgtccgaaatgctgctagtaaaacactacgctcttctaagaaaacttgttgaagggcaagcagtagttcacctcgccagtctgagaagctctcatgagattgagaactatcataaacctcggcttctctttgcagttgcatctttgtaattaaatcctttagagatgagattgtattgatgtaagcttttctctcttctagccaaggttctgaaacctgctgaatagaatggtcctctccatcactatagggagactcagtgagagaaagcacctgcatgccttcattatggacagctctcagtaatccctttattttctttggaaaggaatctgttgcactttcactttcttctcctcggccttctgatgctatgtcaaatccctgactgtgtgtaagataaattccctgaccccagtctgatccagaatcactggagcatatttctctagtctggtaagcatcagaatgtgctagctcaggaattgaggatccctctttacttctcagacactgtatcactgccttcaaggtaccacattcctctttcagtaactgaacggcaacatagtgttccctctttaaggtttcagtttctgaaatatgtctggattccatgtccaaaatttcagcagcatgtagttcttgcatcttctcaattttttcagtaaactgactgattatttcagtaacttcttctgaggaacattcactctgtaaattaatttgtattcctgcatttttaacaagaatttgtggagtctgattgctgctactgatcttcagagtcccatctgtctgggatgcaatgctcttactcagttttataggaagtggctcaaacatgcaggcctttttgctttcttgtacctcagtctcatcttctttttctaaaatggacaatttctcttttgcctctgcgaggtgatccctaacttggcttaagtctttctgaagagatgtcatatttgtttcttttaccaaaagctcttcttgaagtttttcagccttttctttataactggcaagttctgctttggtagccactgattcagctctaagagcctcgagttcattaaaaaatccactttcttcattgctatgaaatagctcagtagttgtcttgagaacttcaacatcttgagggcttcttttcttttctttctctctctgttttttctcattgccctccaatagcttctgtagttctagcagcttcttttctttttctaaaacatttttttctgcaatttctacttgttctttttctaaaatcaaactagtatgcatttcaacaacctggctttctaattctgatattctcaaggttaatgctgatatatctgaccccaactcatcttctcttagttgatttaaattctgaatatttgttctttcaggttctgatgaaattgtttgattatcttgacagaattttgcatattcctgaactgcctcaagttggatttgactgacaagagcagcagccactttttcttcaactattttctgtaggtttacaatcttcttttgaagcatttctgtttcaaactggccttgttcttgcatgtcttttatttgtttataacactgggtaagttctaagtcctttgcactaacagtgctctcaagttgtagcaaccttgtttccaaattaattatggaacctttgccattttcttcaaaagatttgaagtatgtctgattttctagggatttaagagcatcctctgtaaggactacttctagttcaggtttgtctttgctcagatgatctatagccacgttaacactattctctggtatgctttgaatcttttccacactttcacgttctctctttaagctgaataattcctgtgttagctgattcattttaaaattggtttctttaagtacatttttcatgaaggtcatttcttcattagcggtttctacttgctgttccaaggccagcttttcagctataaccacatccaattgatgttttaaactgtctgcttcttctgagagggaatgagcattcattgatgtcttctgtccaatatttgccaattcctgttgaagtttttcaatcacttcattgagctgctctatttcttcttctctatttctcttcacacattcttgatcactcatcaaacattctatttgggtttcaagatcccttatcagttcatttttttcttcaataaccttgttatctgttgtaattttaagttgctgctggagtttcgtaacttgttcatttaattggtcaatttctacctctttttcctgtattatttgagcaaatttcccaaatagcacatgttggtcttgagtagacatggcatcagattcctttatggcaagtcccagtttctccatgtcatccttaaataatttgttttcctgttcaagttcttgtaggcgggtagtagattcctttttctgtatttctaattgcatatgtaattgttgaacttcttcattcttattttccagttcttctctaaactgttctaattgctcttctaagtttgtaatctctttttcctttctgtctatggcatctcgttcagcctgcaattgtacttctagggacaattctggtttagcttctacagctccaaagtgttttcggtcctctaccttttgaaaagtatctgcactcacaagaagcgcctgctccagttctcttactctgaactccagtttctctatttcttcattcctttcttgtatatccctttgaagctgctctttagagagcaaaagctcactgcatttgtctgttttttctttcagatgatttgctaactgttcaacctctctagtttgatgttcactgataggctggaatcgaggaacaaccttaagttgctgttctagtttctgtatttcctgttggaatacatctctctcatgttctctgtcaatggcttgctcatctaaaaattttctcattttttctaactgcttttccaatgcttggttttgctgtcttaaatccattagttcagtatttttttcttgttccagctctataaacctactgacttgttcttccacatctatttctagagctttcacttgtttttgaaggtcatcacgtactttttcagcttgacattgtacttctagtttttccttcattaatttttctgtctcctgtagtaattctgctcctggtgctgcatcgactgcagcatctactagtcgttgttcaactgggcctgcctctgctttcatagcttccttttgtctggacagtaattctctttcttcttggatctgctgttgctctgcctccaattcttgcaacctgttacttgcacataacaactcctgctcaagacgatctattatatcagttttttcctgaatttgcctttcaaaaagagttttttcatctgcatagccatcaatgacgccctcagccttactgagctccacagctagctgttctctggccctggactcctcatgaaggcgctctcgaagttcctcttggcacttaagggactctgttgcttcttgtttctgtctaaatgactcacgcatcaactctgtctgtgtcactttcgcatgttcaagctgactgctagtttcacttatggcttctaggagtttttcaactgctgcttgtagtcgagagctaatgttcagcataagttcttcattttcagggtctatttcagttccagcaaaaccactcctcacaagtcgttgtgacagctctgttccttcctcagttacttttgaccacatgttaatgtcatttcttggcatatcacttccagaataagagggaatggattcatctgtaactcttgtatgttcctcatggacacatgactttacagatgcctctgcttctgacctccaaattaggctggcagatgactggcttttactagatctatctagaatcccaaggacatggcgaccaattgtttcttcaacagctgctgttgtctttacaacttctaagaggatcttcaaaagtctattattagctttctggagtgcatacctttcattagacaaaatctcaggaggcacatcttcaggttttctgtctaattccttttctttaaatgtttgttcttcaacttctccttggttttcatttccattctgggctaattgtctattaagtctcttaatctcttcttgtagctgttcctggtcttctcgctgtctctccatttgccgcatatgtgcttgccttaacaattccgttgcctgttgatgttcttggtattgtcgtacaagttcctgtctcatatcttccaactgttcttcattcaacattagttgtctagaagcatccatgcttgacactgaaatctcatcatgaatagactgtctaactataaatgttttatctttggagaacatttcttctgaaatagtcagcacacagtcctttgattctggtatatcatggggatcactatttgataataaaatttcctttccatgttctcctaactctttactaagtggtttaaattcttctttaaatttcacatccactgtctcaaaagtctgaaaaccaatttgatcctgtgataatttcatttcattaaaataatgttgttcttgctgacacacagcatgtgcttgctttgatgatgcagtattttcttttcccccagatattctagacagttcagtttgttgagcaaatgctatactcattgacacaataaccttagctacttcttcttctaattgttcttggtattgtttttcaagcaacttaacgatatttgtttcctctttcactccaaattcaccagaaaactctattgtaccatcaatattctttttcacacaacttccagggtacattgttctctgtgcatcagattctgtaattaccaccgaatcaacaggtaagcttggcggaaccgtggactcactaacagcttgaagcctcttctgtaaacagtggatctctgcctcatagttttgttcagtttctttcaactgttgctgcaaagaggatatgaggctttctaattcttgaacttgttcttcaagtttagttttttcaagatcttgcagagaagataacttgcttttatgattgacatcaatgtcttccaaattggtcatctgagaatggattgataaaaactctgtttcctcttttggaaggttttcttctccaaattcaagtttcataccatctgtctgctgtccccagatcttgcttagtcgtgtttgaagtaccaagagtttgttgtattcttctgttactttgttgagaagagtgtgcatattttcttgaaagtcttgaacttcatatctataatcttgtaattctggatcttcattttcagaaatgtaatcaccagaattctctttgtcttctgcatttacttcacattttaaagcaggagtataatattcaccaaggacactgcataaagtctgtaaaaaataagaacattcttcagacactgccttttgaagttttccaatgagcagatgtaaaggctttccttcatcacctgtttcttgtgttttcatagtctgtagttctaactggtgtattttctgaagttccttgatcttttcctcttgagcaaaaataagctcttctttaagactgcaaagagctttatctttttcattttccatatattcacgaacctgatccacatgagttgaataaaccagagagaggcaaatgcgttgggcttccatctgtagccttaaatcattctgttctgatttaagtacattgagttctttctgaagtttatcattttcacttggttgagttgctctaagtgatgattcctttgttacagatggtaagtgatccaaaatcaactgttcttgcttactttcttctccaacagtcatattttcaaaagaaactttatcttccaccattatttttgattcttcaccaaaacttttatttactttagaaactgatccttcagcacccctgcttgtcatggtcacaactccatctaataaagagcttacttgagtatcacatgactgtacattttctgccctgttgtggttaataatgatttctagctctctacatctcaatgaaacttgttctttctcttgctttaaagatttaacttcttcatttagaaaactaatctcaccatgtttctgtttcaattgttcagaaagatcagacagtctctgtgacagctctaatttctctcgcttggttacctcaagtttttccatgagttctgttgtatccttttcaacaacctcacccatttccaatgtttctgctacaaaagttttgtcttcatcaaagacagaacttttcattttcactgtagttggatttattctttgcaaatgaagctcttcattaagtgctttaagtttacttttatactctaattcctgtttatttttactgtcttctaaatcatcttttactttgagaaggcaagcatactcctcttgtaactcttgatagttaacttcaaagtttttttcagcaaatgaaaaagtgttcctttgcttttcaatctcttcatttagctgaatacattgttgtttgaggtcctcattttcctctataagtatttctatttctttttcccacacagagtctttggatttggacttaatggagtctaagaaaatcaatctttcttcttggctaacaggagtatgtattttcaacatgtcttcaagggttttcttttcatctttaagaatgctattctctgcttcaagttgtgcaaatttttcttgaagatcattctctttttccttcatctgtttttctaacaattctgttttaagttgtaattcttgaacttcttgttcaagtgtacccttttctttttcttcttgtctgagtatttcaatttctttttgaagttcattgatttgaagagtcatttcttctgactttgaatttacaagagactgctgtaaatcttttagctttgaaatttccaaaattaattgattctgcttagttatcaaattgtccttttcaaactgcatggtttctatcttttgactcatttcattctgtaaaccatctatctgctgtttatagtgaatgcctaaattatctttaagtttttcaatatttattcgatgttcaatttctaaatcttccttcagtttggaaagctcttcttcgtgactaaatagaagctgtgttctcagcctctctaattcagcttcttgtgattcagccattctgtctaacacagcattcttttctttttctaacatttcaagttttatcttgtaatttgtaacttctgcttcatgttttaattctagttcctttctggattcagatgcagaaacaatctcagctttcaaatcttccactgtactaagggacttatgtgcttcattaagtttactttcttgttcagctattgtctgtctagctctctgaatctgttcccttgaaaagctcaattcttcaacaaggtcttcaagctgtctctgtagagcacacttttcttctaaaattagtcctagttcttccttgagtttttccttttgagagttagtatcttgcaattttatattcagttcatttattgccacattcattaactttatctgatcttcattaactgtaatatttgaatatgaccttaaagcattctccatttctcccttatgccgtgttttcatttcctccatctgtgccatgtgttgtcttattaattcttgtttcatttgcactatctgctgcccatacatctcatccagctctgcccggagttgttctaactttctttgtgtttcttgttccattcgttgtactatatcagtttcgaactggctgtctttatgatttctcttctgaagttcttcgactgtccccattaactgttttatttcttcagaagactgtctttctttttgcttagaattagtcagctctaatttcatgttttttatttcttggttcttttgcacaatctgttcttgtaattctcctagtaatttatcagcagttgttaatttatcctttagctcaagagttttcttttcttcttctattatttttgtgtttaattcttcaatgattgtctccttttcctgtatttcttctttatttgagttttctacttttttatcttgttccatttcatatactttaattttctcttgcaagaaactaatttgcattgtgaagtcttctttctttttctgataatcttctaataagtggtcttgttcttcaagctgctgttgatgagtgaggatctgttgtttggcttgtagtaagtctgcagctgtgctactatgagtgctgtttctcagagtttcactagcctgtaattgctgaaattgaatctgtaatttttgactctgttctgtcaactctaaaaattctctcattgtctcatccttttctcttcttgcttgttgtaaattagcagtgagctgggttataatgccatctctttgtttaatggcagcttcaaattcttgtaactgctgcagtccttcagtcccataggtaaccctcatttcttccagctctctgtttagctcttcaatctcatgctgcttcccagccaactcactttccatcatctctagatgagtcggactgtcttgtgctccttgttcagaataagaatcatcaacaccaaattcttcttcccttaataaatttgtaggctttcctgttctcatcacaaaactgcaaccatttacctctgaactgcagtcatctgctgtggttgaaatttcactttccagttccacagagaagccctgctcatgactggttatttctccactatgtagagttctcattattgtagattcaggaatcacagttgattctactctctgagaactatttatgtacatttcattacactgtgattgatcaatattcaaatcatggtgtgctgacacatcatgtttactgcttgacgtttttctcttttttttctgcttcttggaaggactctgcccatccgactgagcttttctttgtcgaaactgggcaagcttggctttgccggcctccagcttcttctgtctctcctcgtcctccatggcctctgcaaggaaggcaggggaaaacaggggttgaggggtggttggggatagaaaggaaaggtcgatttggacggaggtgggacggcaagctccacggcctagagagccgattcggtccggcgctcccccgcccgaagtggaagcagtctccgcgctcactggcggatcgtcctcagccgcacgggaagcgccgtcaccgccgccgccgccgccatcttcgtctccacgta

SEQ ID NO: 14222 - RNA, 13015 nt, Homo sapiens
  source 1..13015: mol_type = other RNA
gctgggattacaggcatgagccaccgcgcccagcccatatacttaagctgacttttaagagattttgaatatatatgtaaaaatcaccatgactggctctatggcaaggtaggtgagactaatatttagagtttttttaaagtgctctcaaagttggatgttctatacctcatacatttttgaaaaatcttttggtcttcaaaatctgggtcttgtgaaatttggatgctcaaaacaaaacaagcctaggcaaaccaacaaactcagctatgataataaaagtttcctattactacaagatgcttgggtgtaaacaaatgatttcttgaaggaagagataaactactcaatgattcaaagtctctgaatcaggagtgaactgaagtgagatagggaaaagaggttttccttccatgaacagggaatccacctttattttaaagtatgacttgttttttgtttttgaacaaagaaaaaataatccttacaaagtattttaaatgggatagtttttttcgatgatacataaaagcacaatatagtagcagggataatggttacattaagtgcttaaagtaagtgcttcctccttaactccacccgatttgcatgccttaccactttcttttttttttttttttctttgagacagggtctcgctctgctgcccaggctggagtgctgcggcacggccttaccactttctgccatgcgctacttaggaatacgttctccagttaggctctgtagactcagagtaccttgcacactggtgctcattgtgcattttgtgtcatcagtccgctgaatgaacatagtaggaaatcatttttgggaggagtgggatctggggtgataaatcatattttcacttaaattatttaaagtcagtttctctgctggttacaagagtttaagctttggctaacttaataattagctcatgcactaaactggaagctttgattatcctaatgagtgtgaaagaatttcaaagaaaggggagctgtgggtctcgcactgtggtgctgccaagatgtggttaaactcagagcacctgactgtatagttccaagtcgtctttgcagtgcctctagccgagtgatataatctgttagggctctgtcaggatcgtaattctgaagctgagaacatgctaaagaaccaggattgaaatcagctggagtgcctgggtacctattctgaaatggtaaaggggacctaatatagtccagatctgatcttgagcgatacgtagtatgtcttggttctccatataactccagcccaccagaagaatgataaaatgagtcagtcttttctgcaccttgattcagtccaaagccatctctgttaatattgatggaaacagaacctgtgactcgatgccaccgtcgaaccaaaaatttcattctggaaattgcaatggatactctgacggccgaccgaaacctggtgaagccctttgggcgattggtgatcacctctagatccgtgaaagctggctgcccccccatccgggcaagcagggccaaggtggcatcttcacattcctggaacccacccagtaacagcagcaggtatttcttctggtaaatgagagcctttcgaaaactttctgccctcaagtatttaccataaattctctttaaagtgacatgttcagaatcagggctcagagtttgaagtaaagagtcatttcttagttcagctttcagtttgtatacttcagcctctgcccttttcaaagatttctggagagtcaatttttctctgttccatacttctttttcagaggcaatgatggcttcaatgttggcaccaccattcaatgaaaacctggaagaattatctctaccagctcctgtctgtcgataccacctgatctgctcttccagcttcataaccatgttccttaagtcattcttctcttcagtcagttgactgatatgccctgtcagctcagcattttgtctcagtagtctttcagtcaatgagccacaagaagtacttggggacaccaagctgggctcttcaccttgctggccagttaatttctgtagttgtaaaataatttcatcaatattttcctgaacccaaatgaaatcttcatcatctgctgtttcaaactgtagtctctcagaggctttctggggtagaacctgtagttttgaagctacacattgaagcttttgtctgatcatttctaattcatgattacagccggttcctcctccattcatttcaatcaatttagcgtagtttgattcttttgtttctccttctattttctgttgaagaacccaatttctagttctatcactggttaagctccacgtggttggctcattaaggttctgatacagaattcttctactttctcgtttttcttctcgttctagttcttgcttctggaattcctgcatgattccttgtagtcgctgtccttcaaggtctaacttataaacttgttgtcttttctcttccagctggcgctgaagatcttccactttggactggagctcatgcatttttttctgtccctcagtgttggcctcctgttctgtctgcagtgttttcctgtgaacctgcctatctttttccatttgctgtcgtgtttgcaaagaatccagtttatatttttcagtctcatttaacaattctactatgcgactgtgtttttcctctagctgtttctgcagctctttcagtaggtcctctgagggcaagggtggccgagactgtccagtaccatcactgctctgcagctgtgcgtgcaattcccgctccctatctagggtactactcatttcccgaattcgaactttctcagattcaagaagtacctgaagctctaagtttcgaccttgttcttctgacaactgggcatcatatagcattctctgtgattctattttttgctgggattcgttcagtagttgtttctgttgttccaaaagtagatttagctgaagattcctttgtttctgactctcaagtgaaaacttcagatcctcaagttcttctttatcccgttcttcactgcgtcccaacttggctttctctttctccaaagcccactggagctctcttgattttttctgttcacttgctaatgtgtcattaagcaaatgtacttcatctgtcttatctttaacttccaacctgaaagcctccaattcttttaggtgtttatgctgtgccttgagtgttgtttctagttccaatttagtttgtgcaagctcactcttcagttcagcaaccaccattttctcagaactcagctgctcctgcagttccgttgctctgtctttcatactgctgagctccacttgcatctccagcatttgagactgcttctgctgtatattatattccaagagttcttggcttggtttctcactctcttgttctcttttcagagtaattttcctaccattcatttgtgcatgcagtgcctgaatttcagataacaaactccttctatctgctttctggaggcattccatagctgcttgatattcaacaccctgttcttgtattctctgttccaaacagtttagtaaaccaactgcatctgtagtacctagagctgtcagctccgtccgaaatgctgctagtaaaacactacgctcttctaagaaaacttgttgaagggcaagcagtagttcacctcgccagtctgagaagctctcatgagattgagaactatcataaacctcggcttctctttgcagttgcatctttgtaattaaatcctttagagatgagattgtattgatgtaagcttttctctcttctagccaaggttctgaaacctgctgaatagaatggtcctctccatcactatagggagactcagtgagagaaagcacctgcatgccttcattatggacagctctcagtaatccctttattttctttggaaaggaatctgttgcactttcactttcttctcctcggccttctgatgctatgtcaaatccctgactgtgtgtaagataaattccctgaccccagtctgatccagaatcactggagcatatttctctagtctggtaagcatcagaatgtgctagctcaggaattgaggatccctctttacttctcagacactgtatcactgccttcaaggtaccacattcctctttcagtaactgaacggcaacatagtgttccctctttaaggtttcagtttctgaaatatgtctggattccatgtccaaaatttcagcagcatgtagttcttgcatcttctcaattttttcagtaaactgactgattatttcagtaacttcttctgaggaacattcactctgtaaattaatttgtattcctgcatttttaacaagaatttgtggagtctgattgctgctactgatcttcagagtcccatctgtctgggatgcaatgctcttactcagttttataggaagtggctcaaacatgcaggcctttttgctttcttgtacctcagtctcatcttctttttctaaaatggacaatttctcttttgcctctgcgaggtgatccctaacttggcttaagtctttctgaagagatgtcatatttgtttcttttaccaaaagctcttcttgaagtttttcagccttttctttataactggcaagttctgctttggtagccactgattcagctctaagagcctcgagttcattaaaaaatccactttcttcattgctatgaaatagctcagtagttgtcttgagaacttcaacatcttgagggcttcttttcttttctttctctctctgttttttctcattgccctccaatagcttctgtagttctagcagcttcttttctttttctaaaacatttttttctgcaatttctacttgttctttttctaaaatcaaactagtatgcatttcaacaacctggctttctaattctgatattctcaaggttaatgctgatatatctgaccccaactcatcttctcttagttgatttaaattctgaatatttgttctttcaggttctgatgaaattgtttgattatcttgacagaattttgcatattcctgaactgcctcaagttggatttgactgacaagagcagcagccactttttcttcaactattttctgtaggtttacaatcttcttttgaagcatttctgtttcaaactggccttgttcttgcatgtcttttatttgtttataacactgggtaagttctaagtcctttgcactaacagtgctctcaagttgtagcaaccttgtttccaaattaattatggaacctttgccattttcttcaaaagatttgaagtatgtctgattttctagggatttaagagcatcctctgtaaggactacttctagttcaggtttgtctttgctcagatgatctatagccacgttaacactattctctggtatgctttgaatcttttccacactttcacgttctctctttaagctgaataattcctgtgttagctgattcattttaaaattggtttctttaagtacatttttcatgaaggtcatttcttcattagcggtttctacttgctgttccaaggccagcttttcagctataaccacatccaattgatgttttaaactgtctgcttcttctgagagggaatgagcattcattgatgtcttctgtccaatatttgccaattcctgttgaagtttttcaatcacttcattgagctgctctatttcttcttctctatttctcttcacacattcttgatcactcatcaaacattctatttgggtttcaagatcccttatcagttcatttttttcttcaataaccttgttatctgttgtaattttaagttgctgctggagtttcgtaacttgttcatttaattggtcaatttctacctctttttcctgtattatttgagcaaatttcccaaatagcacatgttggtcttgagtagacatggcatcagattcctttatggcaagtcccagtttctccatgtcatccttaaataatttgttttcctgttcaagttcttgtaggcgggtagtagattcctttttctgtatttctaattgcatatgtaattgttgaacttcttcattcttattttccagttcttctctaaactgttctaattgctcttctaagtttgtaatctctttttcctttctgtctatggcatctcgttcagcctgcaattgtacttctagggacaattctggtttagcttctacagctccaaagtgttttcggtcctctaccttttgaaaagtatctgcactcacaagaagcgcctgctccagttctcttactctgaactccagtttctctatttcttcattcctttcttgtatatccctttgaagctgctctttagagagcaaaagctcactgcatttgtctgttttttctttcagatgatttgctaactgttcaacctctctagtttgatgttcactgataggctggaatcgaggaacaaccttaagttgctgttctagtttctgtatttcctgttggaatacatctctctcatgttctctgtcaatggcttgctcatctaaaaattttctcattttttctaactgcttttccaatgcttggttttgctgtcttaaatccattagttcagtatttttttcttgttccagctctataaacctactgacttgttcttccacatctatttctagagctttcacttgtttttgaaggtcatcacgtactttttcagcttgacattgtacttctagtttttccttcattaatttttctgtctcctgtagtaattctgctcctggtgctgcatcgactgcagcatctactagtcgttgttcaactgggcctgcctctgctttcatagcttccttttgtctggacagtaattctctttcttcttggatctgctgttgctctgcctccaattcttgcaacctgttacttgcacataacaactcctgctcaagacgatctattatatcagttttttcctgaatttgcctttcaaaaagagttttttcatctgcatagccatcaatgacgccctcagccttactgagctccacagctagctgttctctggccctggactcctcatgaaggcgctctcgaagttcctcttggcacttaagggactctgttgcttcttgtttctgtctaaatgactcacgcatcaactctgtctgtgtcactttcgcatgttcaagctgactgctagtttcacttatggcttctaggagtttttcaactgctgcttgtagtcgagagctaatgttcagcataagttcttcattttcagggtctatttcagttccagcaaaaccactcctcacaagtcgttgtgacagctctgttccttcctcagttacttttgaccacatgttaatgtcatttcttggcatatcacttccagaataagagggaatggattcatctgtaactcttgtatgttcctcatggacacatgactttacagatgcctctgcttctgacctccaaattaggctggcagatgactggcttttactagatctatctagaatcccaaggacatggcgaccaattgtttcttcaacagctgctgttgtctttacaacttctaagaggatcttcaaaagtctattattagctttctggagtgcatacctttcattagacaaaatctcaggaggcacatcttcaggttttctgtctaattccttttctttaaatgtttgttcttcaacttctccttggttttcatttccattctgtgtttgcgtactgctgttgcgcagctcacaacacagcttctctcttccagctaaagacagctgctttagtgcttccagctcctctaaaagcaccctctctctctctgaaaccaggttttcattatctatggaggatctctgggctaattgtctattaagtctcttaatctcttcttgtagctgttcctggtcttctcgctgtctctccatttgccgcatatgtgcttgccttaacaattccgttgcctgttgatgttcttggtattgtcgtacaagttcctgtctcatatcttccaactgttcttcattcaacattagttgtctagaagcatccatgcttgacactgaaatctcatcatgaatagactgtctaactataaatgttttatctttggagaacatttcttctgaaatagtcagcacacagtcctttgattctggtatatcatggggatcactatttgataataaaatttcctttccatgttctcctaactctttactaagtggtttaaattcttctttaaatttcacatccactgtctcaaaagtctgaaaaccaatttgatcctgtgataatttcatttcattaaaataatgttgttcttgctgacacacagcatgtgcttgctttgatgatgcagtattttcttttcccccagatattctagacagttcagtttgttgagcaaatgctatactcattgacacaataaccttagctacttcttcttctaattgttcttggtattgtttttcaagcaacttaacgatatttgtttcctctttcactccaaattcaccagaaaactctattgtaccatcaatattctttttcacacaacttccagggtacattgttctctgtgcatcagattctgtaattaccaccgaatcaacaggtaagcttggcggaaccgtggactcactaacagcttgaagcctcttctgtaaacagtggatctctgcctcatagttttgttcagtttctttcaactgttgctgcaaagaggatatgaggctttctaattcttgaacttgttcttcaagtttagttttttcaagatcttgcagagaagataacttgcttttatgattgacatcaatgtcttccaaattggtcatctgagaatggattgataaaaactctgtttcctcttttggaaggttttcttctccaaattcaagtttcataccatctgtctgctgtccccagatcttgcttagtcgtgtttgaagtaccaagagtttgttgtattcttctgttactttgttgagaagagtgtgcatattttcttgaaagtcttgaacttcatatctataatcttgtaattctggatcttcattttcagaaatgtaatcaccagaattctctttgtcttctgcatttacttcacattttaaagcaggagtataatattcaccaaggacactgcataaagtctgtaaaaaataagaacattcttcagacactgccttttgaagttttccaatgagcagatgtaaaggctttccttcatcacctgtttcttgtgttttcatagtctgtagttctaactggtgtattttctgaagttccttgatcttttcctcttgagcaaaaataagctcttctttaagactgcaaagagctttatctttttcattttccatatattcacgaacctgatccacatgagttgaataaaccagagagaggcaaatgcgttgggcttccatctgtagccttaaatcattctgttctgatttaagtacattgagttctttctgaagtttatcattttcacttggttgagttgctctaagtgatgattcctttgttacagatggtaagtgatccaaaatcaactgttcttgcttactttcttctccaacagtcatattttcaaaagaaactttatcttccaccattatttttgattcttcaccaaaacttttatttactttagaaactgatccttcagcacccctgcttgtcatggtcacaactccatctaataaagagcttacttgagtatcacatgactgtacattttctgccctgttgtggttaataatgatttctagctctctacatctcaatgaaacttgttctttctcttgctttaaagatttaacttcttcatttagaaaactaatctcaccatgtttctgtttcaattgttcagaaagatcagacagtctctgtgacagctctaatttctctcgcttggttacctcaagtttttccatgagttctgttgtatccttttcaacaacctcacccatttccaatgtttctgctacaaaagttttgtcttcatcaaagacagaacttttcattttcactgtagttggatttattctttgcaaatgaagctcttcattaagtgctttaagtttacttttatactctaattcctgtttatttttactgtcttctaaatcatcttttactttgagaaggcaagcatactcctcttgtaactcttgatagttaacttcaaagtttttttcagcaaatgaaaaagtgttcctttgcttttcaatctcttcatttagctgaatacattgttgtttgaggtcctcattttcctctataagtatttctatttctttttcccacacagagtctttggatttggacttaatggagtctaagaaaatcaatctttcttcttggctaacaggagtatgtattttcaacatgtcttcaagggttttcttttcatctttaagaatgctattctctgcttcaagttgtgcaaatttttcttgaagatcattctctttttccttcatctgtttttctaacaattctgttttaagttgtaattcttgaacttcttgttcaagtgtacccttttctttttcttcttgtctgagtatttcaatttctttttgaagttcattgatttgaagagtcatttcttctgactttgaatttacaagagactgctgtaaatcttttagctttgaaatttccaaaattaattgattctgcttagttatcaaattgtccttttcaaactgcatggtttctatcttttgactcatttcattctgtaaaccatctatctgctgtttatagtgaatgcctaaattatctttaagtttttcaatatttattcgatgttcaatttctaaatcttccttcagtttggaaagctcttcttcgtgactaaatagaagctgtgttctcagcctctctaattcagcttcttgtgattcagccattctgtctaacacagcattcttttctttttctaacatttcaagttttatcttgtaatttgtaacttctgcttcatgttttaattctagttcctttctggattcagatgcagaaacaatctcagctttcaaatcttccactgtactaagggacttatgtgcttcattaagtttactttcttgttcagctattgtctgtctagctctctgaatctgttcccttgaaaagctcaattcttcaacaaggtcttcaagctgtctctgtagagcacacttttcttctaaaattagtcctagttcttccttgagtttttccttttgagagttagtatcttgcaattttatattcagttcatttattgccacattcattaactttatctgatcttcattaactgtaatatttgaatatgaccttaaagcattctccatttctcccttatgccgtgttttcatttcctccatctgtgccatgtgttgtcttattaattcttgtttcatttgcactatctgctgcccatacatctcatccagctctgcccggagttgttctaactttctttgtgtttcttgttccattcgttgtactatatcagtttcgaactggctgtctttatgatttctcttctgaagttcttcgactgtccccattaactgttttatttcttcagaagactgtctttctttttgcttagaattagtcagctctaatttcatgttttttatttcttggttcttttgcacaatctgttcttgtaattctcctagtaatttatcagcagttgttaatttatcctttagctcaagagttttcttttcttcttctattatttttgtgtttaattcttcaatgattgtctccttttcctgtatttcttctttatttgagttttctacttttttatcttgttccatttcatatactttaattttctcttgcaagaaactaatttgcattgtgaagtcttctttctttttctgataatcttctaataagtggtcttgttcttcaagctgctgttgatgagtgaggatctgttgtttggcttgtagtaagtctgcagctgtgctactatgagtgctgtttctcagagtttcactagcctgtaattgctgaaattgaatctgtaatttttgactctgttctgtcaactctaaaaattctctcattgtctcatccttttctcttcttgcttgttgtaaattagcagtgagctgggttataatgccatctctttgtttaatggcagcttcaaattcttgtaactgctgcagtccttcagtcccataggtaaccctcatttcttccagctctctgtttagctcttcaatctcatgctgcttcccagccaactcactttccatcatctctagatgagtcggactgtcttgtgctccttgttcagaataagaatcatcaacaccaaattcttcttcccttaataaatttgtaggctttcctgttctcatcacaaaactgcaaccatttacctctgaactgcagtcatctgctgtggttgaaatttcactttccagttccacagagaagccctgctcatgactggttatttctccactatgtagagttctcattattgtagattcaggaatcacagttgattctactctctgagaactatttatgtacatttcattacactgtgattgatcaatattcaaatcatggtgtgctgacacatcatgtttactgcttgacgtttttctcttttttttctgcttcttggaaggactctgcccatccgactgagcttttctttgtcgaaactgggcaagcttggctttgccggcctccagcttcttctgtctctcctcgtcctccatggcctctgcaaggaaggcaggggaaaacaggggttgaggggtggttggggatagaaaggaaaggtcgatttggacggaggtgggacggcaagctccacggcctagagagccgattcggtccggcgctcccccgcccgaagtggaagcagtctccgcgctcactggcggatcgtcctcagccgcacgggaagcgccgtcaccgccgccgccgccgccatcttcgtctccacgta

SEQ ID NO: 14223 - RNA, 7982 nt, Homo sapiens
  source 1..7982: mol_type = other RNA
gctgggattacaggcatgagccaccgcgcccagcccatatacttaagctgacttttaagagattttgaatatatatgtaaaaatcaccatgactggctctatggcaaggtaggtgagactaatatttagagtttttttaaagtgctctcaaagttggatgttctatacctcatacatttttgaaaaatcttttggtcttcaaaatctgggtcttgtgaaatttggatgctcaaaacaaaacaagcctaggcaaaccaacaaactcagctatgataataaaagtttcctattactacaagatgcttgggtgtaaacaaatgatttcttgaaggaagagataaactactcaatgattcaaagtctctgaatcaggagtgaactgaagtgagatagggaaaagaggttttccttccatgaacagggaatccacctttattttaaagtatgacttgttttttgtttttgaacaaagaaaaaataatccttacaaagtattttaaatgggatagtttttttcgatgatacataaaagcacaatatagtagcagggataatggttacattaagtgcttaaagtaagtgcttcctccttaactccacccgatttgcatgccttaccactttcttttttttttttttttctttgagacagggtctcgctctgctgcccaggctggagtgctgcggcacggccttaccactttctgccatgcgctacttaggaatacgttctccagttaggctctgtagactcagagtaccttgcacactggtgctcattgtgcattttgtgtcatcagtccgctgaatgaacatagtaggaaatcatttttgggaggagtgggatctggggtgataaatcatattttcacttaaattatttaaagtcagtttctctgctggttacaagagtttaagctttggctaacttaataattagctcatgcactaaactggaagctttgattatcctaatgagtgtgaaagaatttcaaagaaaggggagctgtgggtctcgcactgtggtgctgccaagatgtggttaaactcagagcacctgactgtatagttccaagtcgtctttgcagtgcctctagccgagtgatataatctgttagggctctgtcaggatcgtaattctgaagctgagaacatgctaaagaaccaggattgaaatcagctggagtgcctgggtacctattctgaaatggtaaaggggacctaatatagtccagatctgatcttgagcgatacgtagtatgtcttggttctccatataactccagcccaccagaagaatgataaaatgagtcagtcttttctgcaccttgattcagtccaaagccatctctgttaatattgatggaaacagaacctgtgactcgatgccaccgtcgaaccaaaaatttcattctggaaattgcaatggatactctgacggccgaccgaaacctggtgaagccctttgggcgattggtgatcacctctagatccgtgaaagctggctgcccccccatccgggcaagcagggccaaggtggcatcttcacattcctggaacccacccagtaacagcagcaggtatttcttctggtaaatgagagcctttcgaaaactttctgccctcaagtatttaccataaattctctttaaagtgacatgttcagaatcagggctcagagtttgaagtaaagagtcatttcttagttcagctttcagtttgtatacttcagcctctgcccttttcaaagatttctggagagtcaatttttctctgttccatacttctttttcagaggcaatgatggcttcaatgttggcaccaccattcaatgaaaacctggaagaattatctctaccagctcctgtctgtcgataccacctgatctgctcttccagcttcataaccatgttccttaagtcattcttctcttcagtcagttgactgatatgccctgtcagctcagcattttgtctcagtagtctttcagtcaatgagccacaagaagtacttggggacaccaagctgggctcttcaccttgctggccagttaatttctgtagttgtaaaataatttcatcaatattttcctgaacccaaatgaaatcttcatcatctgctgtttcaaactgtagtctctcagaggctttctggggtagaacctgtagttttgaagctacacattgaagcttttgtctgatcatttctaattcatgattacagccggttcctcctccattcatttcaatcaatttagcgtagtttgattcttttgtttctccttctattttctgttgaagaacccaatttctagttctatcactggttaagctccacgtggttggctcattaaggttctgatacagaattcttctactttctcgtttttcttctcgttctagttcttgcttctggaattcctgcatgattccttgtagtcgctgtccttcaaggtctaacttataaacttgttgtcttttctcttccagctggcgctgaagatcttccactttggactggagctcatgcatttttttctgtccctcagtgttggcctcctgttctgtctgcagtgttttcctgtgaacctgcctatctttttccatttgctgtcgtgtttgcaaagaatccagtttatatttttcagtctcatttaacaattctactatgcgactgtgtttttcctctagctgtttctgcagctctttcagtaggtcctctgagggcaagggtggccgagactgtccagtaccatcactgctctgcagctgtgcgtgcaattcccgctccctatctagggtactactcatttcccgaattcgaactttctcagattcaagaagtacctgaagctctaagtttcgaccttgttcttctgacaactgggcatcatatagcattctctgtgattctattttttgctgggattcgttcagtagttgtttctgttgttccaaaagtagatttagctgaagattcctttgtttctgactctcaagtgaaaacttcagatcctcaagttcttctttatcccgttcttcactgcgtcccaacttggctttctctttctccaaagcccactggagctctcttgattttttctgttcacttgctaatgtgtcattaagcaaatgtacttcatctgtcttatctttaacttccaacctgaaagcctccaattcttttaggtgtttatgctgtgccttgagtgttgtttctagttccaatttagtttgtgcaagctcactcttcagttcagcaaccaccattttctcagaactcagctgctcctgcagttccgttgctctgtctttcatactgctgagctccacttgcatctccagcatttgagactgcttctgctgtatattatattccaagagttcttggcttggtttctcactctcttgttctcttttcagagtaattttcctaccattcatttgtgcatgcagtgcctgaatttcagataacaaactccttctatctgctttctggaggcattccatagctgcttgatattcaacaccctgttcttgtattctctgttccaaacagtttagtaaaccaactgcatctgtagtacctagagctgtcagctccgtccgaaatgctgctagtaaaacactacgctcttctaagaaaacttgttgaagggcaagcagtagttcacctcgccagtctgagaagctctcatgagattgagaactatcataaacctcggcttctctttgcagttgcatctttgtaattaaatcctttagagatgagattgtattgatgtaagcttttctctcttctagccaaggttctgaaacctgctgaatagaatggtcctctccatcactatagggagactcagtgagagaaagcacctgcatgccttcattatggacagctctcagtaatccctttattttctttggaaaggaatctgttgcactttcactttcttctcctcggccttctgatgctatgtcaaatccctgactgtgtgtaagataaattccctgaccccagtctgatccagaatcactggagcatatttctctagtctggtaagcatcagaatgtgctagctcaggaattgaggatccctctttacttctcagacactgtatcactgccttcaaggtaccacattcctctttcagtaactgaacggcaacatagtgttccctctttaaggtttcagtttctgaaatatgtctggattccatgtccaaaatttcagcagcatgtagttcttgcatcttctcaattttttcagtaaactgactgattatttcagtaacttcttctgaggaacattcactctgtaaattaatttgtattcctgcatttttaacaagaatttgtggagtctgattgctgctactgatcttcagagtcccatctgtctgggatgcaatgctcttactcagttttataggaagtggctcaaacatgcaggcctttttgctttcttgtacctcagtctcatcttctttttctaaaatggacaatttctcttttgcctctgcgaggtgatccctaacttggcttaagtctttctgaagagatgtcatatttgtttcttttaccaaaagctcttcttgaagtttttcagccttttctttataactggcaagttctgctttggtagccactgattcagctctaagagcctcgagttcattaaaaaatccactttcttcattgctatgaaatagctcagtagttgtcttgagaacttcaacatcttgagggcttcttttcttttctttctctctctgttttttctcattgccctccaatagcttctgtagttctagcagcttcttttctttttctaaaacatttttttctgcaatttctacttgttctttttctaaaatcaaactagtatgcatttcaacaacctggctttctaattctgatattctcaaggttaatgctgatatatctgaccccaactcatcttctcttagttgatttaaattctgaatatttgttctttcaggttctgatgaaattgtttgattatcttgacagaattttgcatattcctgaactgcctcaagttggatttgactgacaagagcagcagccactttttcttcaactattttctgtaggtttacaatcttcttttgaagcatttctgtttcaaactggccttgttcttgcatgtcttttatttgtttataacactgggtaagttctaagtcctttgcactaacagtgctctcaagttgtagcaaccttgtttccaaattaattatggaacctttgccattttcttcaaaagatttgaagtatgtctgattttctagggatttaagagcatcctctgtaaggactacttctagttcaggtttgtctttgctcagatgatctatagccacgttaacactattctctggtatgctttgaatcttttccacactttcacgttctctctttaagctgaataattcctgtgttagctgattcattttaaaattggtttctttaagtacatttttcatgaaggtcatttcttcattagcggtttctacttgctgttccaaggccagcttttcagctataaccacatccaattgatgttttaaactgtctgcttcttctgagagggaatgagcattcattgatgtcttctgtccaatatttgccaattcctgttgaagtttttcaatcacttcattgagctgctctatttcttcttctctatttctcttcacacattcttgatcactcatcaaacattctatttgggtttcaagatcccttatcagttcatttttttcttcaataaccttgttatctgttgtaattttaagttgctgctggagtttcgtaacttgttcatttaattggtcaatttctacctctttttcctgtattatttgagcaaatttcccaaatagcacatgttggtcttgagtagacatggcatcagattcctttatggcaagtcccagtttctccatgtcatccttaaataatttgttttcctgttcaagttcttgtaggcgggtagtagattcctttttctgtatttctaattgcatatgtaattgttgaacttcttcattcttattttccagttcttctctaaactgttctaattgctcttctaagtttgtaatctctttttcctttctgtctatggcatctcgttcagcctgcaattgtacttctagggacaattctggtttagcttctacagctccaaagtgttttcggtcctctaccttttgaaaagtatctgcactcacaagaagcgcctgctccagttctcttactctgaactccagtttctctatttcttcattcctttcttgtatatccctttgaagctgctctttagagagcaaaagctcactgcatttgtctgttttttctttcagatgatttgctaactgttcaacctctctagtttgatgttcactgataggctggaatcgaggaacaaccttaagttgctgttctagtttctgtatttcctgttggaatacatctctctcatgttctctgtcaatggcttgctcatctaaaaattttctcattttttctaactgcttttccaatgcttggttttgctgtcttaaatccattagttcagtatttttttcttgttccagctctataaacctactgacttgttcttccacatctatttctagagctttcacttgtttttgaaggtcatcacgtactttttcagcttgacattgtacttctagtttttccttcattaatttttctgtctcctgtagtaattctgctcctggtgctgcatcgactgcagcatctactagtcgttgttcaactgggcctgcctctgctttcatagcttccttttgtctggacagtaattctctttcttcttggatctgctgttgctctgcctccaattcttgcaacctgttacttgcacataacaactcctgctcaagacgatctattatatcagttttttcctgaatttgcctttcaaaaagagttttttcatctgcatagccatcaatgacgccctcagccttactgagctccacagctagctgttctctggccctggactcctcatgaaggcgctctcgaagttcctcttggcacttaagggactctgttgcttcttgtttctgtctaaatgactcacgcatcaactctgtctgtgtcactttcgcatgttcaagtgaataaggaggggtaggcagtgaaattttagaaataagctttaatatatgcccgtttcttttatgaataaaatggaaaatagaagtattaacaattactgagttattttcatccaaatgttcacaaagaggaaaaggatgtggtaaaggcacgcgagattcaacctcataaatgtcttcatcttgctcttctaaccacgagccactgactttgacagttgccaaataggtgctataagaatccatcccagaagatacagctgccgagattcctaatttgctttatcaattttctaatacattaaaaagttctttttagtttatcaagatctaccatagcagtataaaaagtttcttttttagcactatcaaataaatgttataaaattaattcatacaactgcacaataaaaggaaggggaaagtccaggaaaaaaactacaaatctaaaaaaacttaggtctctatcaatcttgatgccccctcaaaaaaacccaaaccaaaacaaaaaccaaaaaaaatcaaaaaacaaaaataaaagcaagcaaacaaaaacaccttttaaactagcataattaagtccttgaagagaagaataaaaatataaacatctaattagacgagcaataaaactgcttttaatatcagcgatgtctgtagtaataagtaagccttcaaagcagaacctggcagggaaggtcaagtttgaaatctccatagcagcagtcttgagaaatgcagttgtaacattatttctcttgctcttgctgcttcactctattcaaaaggaaaagctcttct

SEQ ID NO: 14224 - RNA, 13072 nt, Homo sapiens
  source 1..13072: mol_type = other RNA
gctgggattacaggcatgagccaccgcgcccagcccatatacttaagctgacttttaagagattttgaatatatatgtaaaaatcaccatgactggctctatggcaaggtaggtgagactaatatttagagtttttttaaagtgctctcaaagttggatgttctatacctcatacatttttgaaaaatcttttggtcttcaaaatctgggtcttgtgaaatttggatgctcaaaacaaaacaagcctaggcaaaccaacaaactcagctatgataataaaagtttcctattactacaagatgcttgggtgtaaacaaatgatttcttgaaggaagagataaactactcaatgattcaaagtctctgaatcaggagtgaactgaagtgagatagggaaaagaggttttccttccatgaacagggaatccacctttattttaaagtatgacttgttttttgtttttgaacaaagaaaaaataatccttacaaagtattttaaatgggatagtttttttcgatgatacataaaagcacaatatagtagcagggataatggttacattaagtgcttaaagtaagtgcttcctccttaactccacccgatttgcatgccttaccactttcttttttttttttttttctttgagacagggtctcgctctgctgcccaggctggagtgctgcggcacggccttaccactttctgccatgcgctacttaggaatacgttctccagttaggctctgtagactcagagtaccttgcacactggtgctcattgtgcattttgtgtcatcagtccgctgaatgaacatagtaggaaatcatttttgggaggagtgggatctggggtgataaatcatattttcacttaaattatttaaagtcagtttctctgctggttacaagagtttaagctttggctaacttaataattagctcatgcactaaactggaagctttgattatcctaatgagtgtgaaagaatttcaaagaaaggggagctgtgggtctcgcactgtggtgctgccaagatgtggttaaactcagagcacctgactgtatagttccaagtcgtctttgcagtgcctctagccgagtgatataatctgttagggctctgtcaggatcgtaattctgaagctgagaacatgctaaagaaccaggattgaaatcagctggagtgcctgggtacctattctgaaatggtaaaggggacctaatatagtccagatctgatcttgagcgatacgtagtatgtcttggttctccatataactccagcccaccagaagaatgataaaatgagtcagtcttttctgcaccttgattcagtccaaagccatctctgttaatattgatggaaacagaacctgtgactcgatgccaccgtcgaaccaaaaatttcattctggaaattgcaatggatactctgacggccgaccgaaacctggtgaagccctttgggcgattggtgatcacctctagatccgtgaaagctggctgcccccccatccgggcaagcagggccaaggtggcatcttcacattcctggaacccacccagtaacagcagcaggtatttcttctggtaaatgagagcctttcgaaaactttctgccctcaagtatttaccataaattctctttaaagtgacatgttcagaatcagggctcagagtttgaagtaaagagtcatttcttagttcagctttcagtttgtatacttcagcctctgcccttttcaaagatttctggagagtcaatttttctctgttccatacttctttttcagaggcaatgatggcttcaatgttggcaccaccattcaatgaaaacctggaagaattatctctaccagctcctgtctgtcgataccacctgatctgctcttccagcttcataaccatgttccttaagtcattcttctcttcagtcagttgactgatatgccctgtcagctcagcattttgtctcagtagtctttcagtcaatgagccacaagaagtacttggggacaccaagctgggctcttcaccttgctggccagttaatttctgtagttgtaaaataatttcatcaatattttcctgaacccaaatgaaatcttcatcatctgctgtttcaaactgtagtctctcagaggctttctggggtagaacctgtagttttgaagctacacattgaagcttttgtctgatcatttctaattcatgattacagccggttcctcctccattcatttcaatcaatttagcgtagtttgattcttttgtttctccttctattttctgttgaagaacccaatttctagttctatcactggttaagctccacgtggttggctcattaaggttctgatacagaattcttctactttctcgtttttcttctcgttctagttcttgcttctggaattcctgcatgattccttgtagtcgctgtccttcaaggtctaacttataaacttgttgtcttttctcttccagctggcgctgaagatcttccactttggactggagctcatgcatttttttctgtccctcagtgttggcctcctgttctgtctgcagtgttttcctgtgaacctgcctatctttttccatttgctgtcgtgtttgcaaagaatccagtttatatttttcagtctcatttaacaattctactatgcgactgtgtttttcctctagctgtttctgcagctctttcagtaggtcctctgagggcaagggtggccgagactgtccagtaccatcactgctctgcagctgtgcgtgcaattcccgctccctatctagggtactactcatttcccgaattcgaactttctcagattcaagaagtacctgaagctctaagtttcgaccttgttcttctgacaactgggcatcatatagcattctctgtgattctattttttgctgggattcgttcagtagttgtttctgttgttccaaaagtagatttagctgaagattcctttgtttctgactctcaagtgaaaacttcagatcctcaagttcttctttatcccgttcttcactgcgtcccaacttggctttctctttctccaaagcccactggagctctcttgattttttctgttcacttgctaatgtgtcattaagcaaatgtacttcatctgtcttatctttaacttccaacctgaaagcctccaattcttttaggtgtttatgctgtgccttgagtgttgtttctagttccaatttagtttgtgcaagctcactcttcagttcagcaaccaccattttctcagaactcagctgctcctgcagttccgttgctctgtctttcatactgctgagctccacttgcatctccagcatttgagactgcttctgctgtatattatattccaagagttcttggcttggtttctcactctcttgttctcttttcagagtaattttcctaccattcatttgtgcatgcagtgcctgaatttcagataacaaactccttctatctgctttctggaggcattccatagctgcttgatattcaacaccctgttcttgtattctctgttccaaacagtttagtaaaccaactgcatctgtagtacctagagctgtcagctccgtccgaaatgctgctagtaaaacactacgctcttctaagaaaacttgttgaagggcaagcagtagttcacctcgccagtctgagaagctctcatgagattgagaactatcataaacctcggcttctctttgcagttgcatctttgtaattaaatcctttagagatgagattgtattgatgtaagcttttctctcttctagccaaggttctgaaacctgctgaatagaatggtcctctccatcactatagggagactcagtgagagaaagcacctgcatgccttcattatggacagctctcagtaatccctttattttctttggaaaggaatctgttgcactttcactttcttctcctcggccttctgatgctatgtcaaatccctgactgtgtgtaagataaattccctgaccccagtctgatccagaatcactggagcatatttctctagtctggtaagcatcagaatgtgctagctcaggaattgaggatccctctttacttctcagacactgtatcactgccttcaaggtaccacattcctctttcagtaactgaacggcaacatagtgttccctctttaaggtttcagtttctgaaatatgtctggattccatgtccaaaatttcagcagcatgtagttcttgcatcttctcaattttttcagtaaactgactgattatttcagtaacttcttctgaggaacattcactctgtaaattaatttgtattcctgcatttttaacaagaatttgtggagtctgattgctgctactgatcttcagagtcccatctgtctgggatgcaatgctcttactcagttttataggaagtggctcaaacatgcaggcctttttgctttcttgtacctcagtctcatcttctttttctaaaatggacaatttctcttttgcctctgcgaggtgatccctaacttggcttaagtctttctgaagagatgtcatatttgtttcttttaccaaaagctcttcttgaagtttttcagccttttctttataactggcaagttctgctttggtagccactgattcagctctaagagcctcgagttcattaaaaaatccactttcttcattgctatgaaatagctcagtagttgtcttgagaacttcaacatcttgagggcttcttttcttttctttctctctctgttttttctcattgccctccaatagcttctgtagttctagcagcttcttttctttttctaaaacatttttttctgcaatttctacttgttctttttctaaaatcaaactagtatgcatttcaacaacctggctttctaattctgatattctcaaggttaatgctgatatatctgaccccaactcatcttctcttagttgatttaaattctgaatatttgttctttcaggttctgatgaaattgtttgattatcttgacagaattttgcatattcctgaactgcctcaagttggatttgactgacaagagcagcagccactttttcttcaactattttctgtaggtttacaatcttcttttgaagcatttctgtttcaaactggccttgttcttgcatgtcttttatttgtttataacactgggtaagttctaagtcctttgcactaacagtgctctcaagttgtagcaaccttgtttccaaattaattatggaacctttgccattttcttcaaaagatttgaagtatgtctgattttctagggatttaagagcatcctctgtaaggactacttctagttcaggtttgtctttgctcagatgatctatagccacgttaacactattctctggtatgctttgaatcttttccacactttcacgttctctctttaagctgaataattcctgtgttagctgattcattttaaaattggtttctttaagtacatttttcatgaaggtcatttcttcattagcggtttctacttgctgttccaaggccagcttttcagctataaccacatccaattgatgttttaaactgtctgcttcttctgagagggaatgagcattcattgatgtcttctgtccaatatttgccaattcctgttgaagtttttcaatcacttcattgagctgctctatttcttcttctctatttctcttcacacattcttgatcactcatcaaacattctatttgggtttcaagatcccttatcagttcatttttttcttcaataaccttgttatctgttgtaattttaagttgctgctggagtttcgtaacttgttcatttaattggtcaatttctacctctttttcctgtattatttgagcaaatttcccaaatagcacatgttggtcttgagtagacatggcatcagattcctttatggcaagtcccagtttctccatgtcatccttaaataatttgttttcctgttcaagttcttgtaggcgggtagtagattcctttttctgtatttctaattgcatatgtaattgttgaacttcttcattcttattttccagttcttctctaaactgttctaattgctcttctaagtttgtaatctctttttcctttctgtctatggcatctcgttcagcctgcaattgtacttctagggacaattctggtttagcttctacagctccaaagtgttttcggtcctctaccttttgaaaagtatctgcactcacaagaagcgcctgctccagttctcttactctgaactccagtttctctatttcttcattcctttcttgtatatccctttgaagctgctctttagagagcaaaagctcactgcatttgtctgttttttctttcagatgatttgctaactgttcaacctctctagtttgatgttcactgataggctggaatcgaggaacaaccttaagttgctgttctagtttctgtatttcctgttggaatacatctctctcatgttctctgtcaatggcttgctcatctaaaaattttctcattttttctaactgcttttccaatgcttggttttgctgtcttaaatccattagttcagtatttttttcttgttccagctctataaacctactgacttgttcttccacatctatttctagagctttcacttgtttttgaaggtcatcacgtactttttcagcttgacattgtacttctagtttttccttcattaatttttctgtctcctgtagtaattgttgttcaactgggcctgcctctgctttcatagcttccttttgtctggacagtaattctctttcttcttggatctgctgttgctctgcctccaattcttgcaacctgttacttgcacataacaactcctgctcaagacgatctattatatcagttttttcctgaatttgcctttcaaaaagagttttttcatctgcatagccatcaatgacgccctcagccttactgagctccacagctagctgttctctggccctggactcctcatgaaggcgctctcgaagttcctcttggcacttaagggactctgttgcttcttgtttctgtctaaatgactcacgcatcaactctgtctgtgtcactttcgcatgttcaagctgactgctagtttcacttatggcttctaggagtttttcaactgctgcttgtagtcgagagctaatgttcagcataagttcttcattttcagggtctatttcagttccagcaaaaccactcctcacaagtcgttgtgacagctctgttccttcctcagttacttttgaccacatgttaatgtcatttcttggcatatcacttccagaataagagggaatggattcatctgtaactcttgtatgttcctcatggacacatgactttacagatgcctctgcttctgacctccaaattaggctggcagatgactggcttttactagatctatctagaatcccaaggacatggcgaccaattgtttcttcaacagctgctgttgtctttacaacttctaagaggatcttcaaaagtctattattagctttctggagtgcatacactgtctttcttgtttgagttccatactgactgcgttccatactgatgatccaatggggaagccaaaatcttaggggccaaattcctccatgcaagctttcattagacaaaatctcaggaggcacatcttcaggttttctgtctaattccttttctttaaatgtttgttcttcaacttctccttggttttcatttccattctgtgtttgcgtactgctgttgcgcagctcacaacacagcttctctcttccagctaaagacagctgctttagtgcttccagctcctctaaaagcaccctctctctctctgaaaccaggttttcattatctatggaggatctctgggctaattgtctattaagtctcttaatctcttcttgtagctgttcctggtcttctcgctgtctctccatttgccgcatatgtgcttgccttaacaattccgttgcctgttgatgttcttggtattgtcgtacaagttcctgtctcatatcttccaactgttcttcattcaacattagttgtctagaagcatccatgcttgacactgaaatctcatcatgaatagactgtctaactataaatgttttatctttggagaacatttcttctgaaatagtcagcacacagtcctttgattctggtatatcatggggatcactatttgataataaaatttcctttccatgttctcctaactctttactaagtggtttaaattcttctttaaatttcacatccactgtctcaaaagtctgaaaaccaatttgatcctgtgataatttcatttcattaaaataatgttgttcttgctgacacacagcatgtgcttgctttgatgatgcagtattttcttttcccccagatattctagacagttcagtttgttgagcaaatgctatactcattgacacaataaccttagctacttcttcttctaattgttcttggtattgtttttcaagcaacttaacgatatttgtttcctctttcactccaaattcaccagaaaactctattgtaccatcaatattctttttcacacaacttccagggtacattgttctctgtgcatcagattctgtaattaccaccgaatcaacaggtaagcttggcggaaccgtggactcactaacagcttgaagcctcttctgtaaacagtggatctctgcctcatagttttgttcagtttctttcaactgttgctgcaaagaggatatgaggctttctaattcttgaacttgttcttcaagtttagttttttcaagatcttgcagagaagataacttgcttttatgattgacatcaatgtcttccaaattggtcatctgagaatggattgataaaaactctgtttcctcttttggaaggttttcttctccaaattcaagtttcataccatctgtctgctgtccccagatcttgcttagtcgtgtttgaagtaccaagagtttgttgtattcttctgttactttgttgagaagagtgtgcatattttcttgaaagtcttgaacttcatatctataatcttgtaattctggatcttcattttcagaaatgtaatcaccagaattctctttgtcttctgcatttacttcacattttaaagcaggagtataatattcaccaaggacactgcataaagtctgtaaaaaataagaacattcttcagacactgccttttgaagttttccaatgagcagatgtaaaggctttccttcatcacctgtttcttgtgttttcatagtctgtagttctaactggtgtattttctgaagttccttgatcttttcctcttgagcaaaaataagctcttctttaagactgcaaagagctttatctttttcattttccatatattcacgaacctgatccacatgagttgaataaaccagagagaggcaaatgcgttgggcttccatctgtagccttaaatcattctgttctgatttaagtacattgagttctttctgaagtttatcattttcacttggttgagttgctctaagtgatgattcctttgttacagatggtaagtgatccaaaatcaactgttcttgcttactttcttctccaacagtcatattttcaaaagaaactttatcttccaccattatttttgattcttcaccaaaacttttatttactttagaaactgatccttcagcacccctgcttgtcatggtcacaactccatctaataaagagcttacttgagtatcacatgactgtacattttctgccctgttgtggttaataatgatttctagctctctacatctcaatgaaacttgttctttctcttgctttaaagatttaacttcttcatttagaaaactaatctcaccatgtttctgtttcaattgttcagaaagatcagacagtctctgtgacagctctaatttctctcgcttggttacctcaagtttttccatgagttctgttgtatccttttcaacaacctcacccatttccaatgtttctgctacaaaagttttgtcttcatcaaagacagaacttttcattttcactgtagttggatttattctttgcaaatgaagctcttcattaagtgctttaagtttacttttatactctaattcctgtttatttttactgtcttctaaatcatcttttactttgagaaggcaagcatactcctcttgtaactcttgatagttaacttcaaagtttttttcagcaaatgaaaaagtgttcctttgcttttcaatctcttcatttagctgaatacattgttgtttgaggtcctcattttcctctataagtatttctatttctttttcccacacagagtctttggatttggacttaatggagtctaagaaaatcaatctttcttcttggctaacaggagtatgtattttcaacatgtcttcaagggttttcttttcatctttaagaatgctattctctgcttcaagttgtgcaaatttttcttgaagatcattctctttttccttcatctgtttttctaacaattctgttttaagttgtaattcttgaacttcttgttcaagtgtacccttttctttttcttcttgtctgagtatttcaatttctttttgaagttcattgatttgaagagtcatttcttctgactttgaatttacaagagactgctgtaaatcttttagctttgaaatttccaaaattaattgattctgcttagttatcaaattgtccttttcaaactgcatggtttctatcttttgactcatttcattctgtaaaccatctatctgctgtttatagtgaatgcctaaattatctttaagtttttcaatatttattcgatgttcaatttctaaatcttccttcagtttggaaagctcttcttcgtgactaaatagaagctgtgttctcagcctctctaattcagcttcttgtgattcagccattctgtctaacacagcattcttttctttttctaacatttcaagttttatcttgtaatttgtaacttctgcttcatgttttaattctagttcctttctggattcagatgcagaaacaatctcagctttcaaatcttccactgtactaagggacttatgtgcttcattaagtttactttcttgttcagctattgtctgtctagctctctgaatctgttcccttgaaaagctcaattcttcaacaaggtcttcaagctgtctctgtagagcacacttttcttctaaaattagtcctagttcttccttgagtttttccttttgagagttagtatcttgcaattttatattcagttcatttattgccacattcattaactttatctgatcttcattaactgtaatatttgaatatgaccttaaagcattctccatttctcccttatgccgtgttttcatttcctccatctgtgccatgtgttgtcttattaattcttgtttcatttgcactatctgctgcccatacatctcatccagctctgcccggagttgttctaactttctttgtgtttcttgttccattcgttgtactatatcagtttcgaactggctgtctttatgatttctcttctgaagttcttcgactgtccccattaactgttttatttcttcagaagactgtctttctttttgcttagaattagtcagctctaatttcatgttttttatttcttggttcttttgcacaatctgttcttgtaattctcctagtaatttatcagcagttgttaatttatcctttagctcaagagttttcttttcttcttctattatttttgtgtttaattcttcaatgattgtctccttttcctgtatttcttctttatttgagttttctacttttttatcttgttccatttcatatactttaattttctcttgcaagaaactaatttgcattgtgaagtcttctttctttttctgataatcttctaataagtggtcttgttcttcaagctgctgttgatgagtgaggatctgttgtttggcttgtagtaagtctgcagctgtgctactatgagtgctgtttctcagagtttcactagcctgtaattgctgaaattgaatctgtaatttttgactctgttctgtcaactctaaaaattctctcattgtctcatccttttctcttcttgcttgttgtaaattagcagtgagctgggttataatgccatctctttgtttaatggcagcttcaaattcttgtaactgctgcagtccttcagtcccataggtaaccctcatttcttccagctctctgtttagctcttcaatctcatgctgcttcccagccaactcactttccatcatctctagatgagtcggactgtcttgtgctccttgttcagaataagaatcatcaacaccaaattcttcttcccttaataaatttgtaggctttcctgttctcatcacaaaactgcaaccatttacctctgaactgcagtcatctgctgtggttgaaatttcactttccagttccacagagaagccctgctcatgactggttatttctccactatgtagagttctcattattgtagattcaggaatcacagttgattctactctctgagaactatttatgtacatttcattacactgtgattgatcaatattcaaatcatggtgtgctgacacatcatgtttactgcttgacgtttttctcttttttttctgcttcttggaaggactctgcccatccgactgagcttttctttgtcgaaactgggcaagcttggctttgccggcctccagcttcttctgtctctcctcgtcctccatggcctctgcaaggaaggcaggggaaaacaggggttgaggggtggttggggatagaaaggaaaggtcgatttggacggaggtgggacggcaagctccacggcctagagagccgattcggtccggcgctcccccgcccgaagtggaagcagtctccgcgctcactggcggatcgtcctcagccgcacgggaagcgccgtcaccgccgccgccgccgccatcttcgtctccacgta

SEQ ID NO: 14225 - RNA, 12835 nt, Homo sapiens
  source 1..12835: mol_type = other RNA
gctgggattacaggcatgagccaccgcgcccagcccatatacttaagctgacttttaagagattttgaatatatatgtaaaaatcaccatgactggctctatggcaaggtaggtgagactaatatttagagtttttttaaagtgctctcaaagttggatgttctatacctcatacatttttgaaaaatcttttggtcttcaaaatctgggtcttgtgaaatttggatgctcaaaacaaaacaagcctaggcaaaccaacaaactcagctatgataataaaagtttcctattactacaagatgcttgggtgtaaacaaatgatttcttgaaggaagagataaactactcaatgattcaaagtctctgaatcaggagtgaactgaagtgagatagggaaaagaggttttccttccatgaacagggaatccacctttattttaaagtatgacttgttttttgtttttgaacaaagaaaaaataatccttacaaagtattttaaatgggatagtttttttcgatgatacataaaagcacaatatagtagcagggataatggttacattaagtgcttaaagtaagtgcttcctccttaactccacccgatttgcatgccttaccactttcttttttttttttttttctttgagacagggtctcgctctgctgcccaggctggagtgctgcggcacggccttaccactttctgccatgcgctacttaggaatacgttctccagttaggctctgtagactcagagtaccttgcacactggtgctcattgtgcattttgtgtcatcagtccgctgaatgaacatagtaggaaatcatttttgggaggagtgggatctggggtgataaatcatattttcacttaaattatttaaagtcagtttctctgctggttacaagagtttaagctttggctaacttaataattagctcatgcactaaactggaagctttgattatcctaatgagtgtgaaagaatttcaaagaaaggggagctgtgggtctcgcactgtggtgctgccaagatgtggttaaactcagagcacctgactgtatagttccaagtcgtctttgcagtgcctctagccgagtgatataatctgttagggctctgtcaggatcgtaattctgaagctgagaacatgctaaagaaccaggattgaaatcagctggagtgcctgggtacctattctgaaatggtaaaggggacctaatatagtccagatctgatcttgagcgatacgtagtatgtcttggttctccatataactccagcccaccagaagaatgataaaatgagtcagtcttttctgcaccttgattcagtccaaagccatctctgttaatattgatggaaacagaacctgtgactcgatgccaccgtcgaaccaaaaatttcattctggaaattgcaatggatactctgacggccgaccgaaacctggtgaagccctttgggcgattggtgatcacctctagatccgtgaaagctggctgcccccccatccgggcaagcagggccaaggtggcatcttcacattcctggaacccacccagtaacagcagcaggtatttcttctggtaaatgagagcctttcgaaaactttctgccctcaagtatttaccataaattctctttaaagtgacatgttcagaatcagggctcagagtttgaagtaaagagtcatttcttagttcagctttcagtttgtatacttcagcctctgcccttttcaaagatttctggagagtcaatttttctctgttccatacttctttttcagaggcaatgatggcttcaatgttggcaccaccattcaatgaaaacctggaagaattatctctaccagctcctgtctgtcgataccacctgatctgctcttccagcttcataaccatgttccttaagtcattcttctcttcagtcagttgactgatatgccctgtcagctcagcattttgtctcagtagtctttcagtcaatgagccacaagaagtacttggggacaccaagctgggctcttcaccttgctggccagttaatttctgtagttgtaaaataatttcatcaatattttcctgaacccaaatgaaatcttcatcatctgctgtttcaaactgtagtctctcagaggctttctggggtagaacctgtagttttgaagctacacattgaagcttttgtctgatcatttctaattcatgattacagccggttcctcctccattcatttcaatcaatttagcgtagtttgattcttttgtttctccttctattttctgttgaagaacccaatttctagttctatcactggttaagctccacgtggttggctcattaaggttctgatacagaattcttctactttctcgtttttcttctcgttctagttcttgcttctggaattcctgcatgattccttgtagtcgctgtccttcaaggtctaacttataaacttgttgtcttttctcttccagctggcgctgaagatcttccactttggactggagctcatgcatttttttctgtccctcagtgttggcctcctgttctgtctgcagtgttttcctgtgaacctgcctatctttttccatttgctgtcgtgtttgcaaagaatccagtttatatttttcagtctcatttaacaattctactatgcgactgtgtttttcctctagctgtttctgcagctctttcagtaggtcctctgagggcaagggtggccgagactgtccagtaccatcactgctctgcagctgtgcgtgcaattcccgctccctatctagggtactactcatttcccgaattcgaactttctcagattcaagaagtacctgaagctctaagtttcgaccttgttcttctgacaactgggcatcatatagcattctctgtgattctattttttgctgggattcgttcagtagttgtttctgttgttccaaaagtagatttagctgaagattcctttgtttctgactctcaagtgaaaacttcagatcctcaagttcttctttatcccgttcttcactgcgtcccaacttggctttctctttctccaaagcccactggagctctcttgattttttctgttcacttgctaatgtgtcattaagcaaatgtacttcatctgtcttatctttaacttccaacctgaaagcctccaattcttttaggtgtttatgctgtgccttgagtgttgtttctagttccaatttagtttgtgcaagctcactcttcagttcagcaaccaccattttctcagaactcagctgctcctgcagttccgttgctctgtctttcatactgctgagctccacttgcatctccagcatttgagactgcttctgctgtatattatattccaagagttcttggcttggtttctcactctcttgttctcttttcagagtaattttcctaccattcatttgtgcatgcagtgcctgaatttcagataacaaactccttctatctgctttctggaggcattccatagctgcttgatattcaacaccctgttcttgtattctctgttccaaacagtttagtaaaccaactgcatctgtagtacctagagctgtcagctccgtccgaaatgctgctagtaaaacactacgctcttctaagaaaacttgttgaagggcaagcagtagttcacctcgccagtctgagaagctctcatgagattgagaactatcataaacctcggcttctctttgcagttgcatctttgtaattaaatcctttagagatgagattgtattgatgtaagcttttctctcttctagccaaggttctgaaacctgctgaatagaatggtcctctccatcactatagggagactcagtgagagaaagcacctgcatgccttcattatggacagctctcagtaatccctttattttctttggaaaggaatctgttgcactttcactttcttctcctcggccttctgatgctatgtcaaatccctgactgtgtgtaagataaattccctgaccccagtctgatccagaatcactggagcatatttctctagtctggtaagcatcagaatgtgctagctcaggaattgaggatccctctttacttctcagacactgtatcactgccttcaaggtaccacattcctctttcagtaactgaacggcaacatagtgttccctctttaaggtttcagtttctgaaatatgtctggattccatgtccaaaatttcagcagcatgtagttcttgcatcttctcaattttttcagtaaactgactgattatttcagtaacttcttctgaggaacattcactctgtaaattaatttgtattcctgcatttttaacaagaatttgtggagtctgattgctgctactgatcttcagagtcccatctgtctgggatgcaatgctcttactcagttttataggaagtggctcaaacatgcaggcctttttgctttcttgtacctcagtctcatcttctttttctaaaatggacaatttctcttttgcctctgcgaggtgatccctaacttggcttaagtctttctgaagagatgtcatatttgtttcttttaccaaaagctcttcttgaagtttttcagccttttctttataactggcaagttctgctttggtagccactgattcagctctaagagcctcgagttcattaaaaaatccactttcttcattgctatgaaatagctcagtagttgtcttgagaacttcaacatcttgagggcttcttttcttttctttctctctctgttttttctcattgccctccaatagcttctgtagttctagcagcttcttttctttttctaaaacatttttttctgcaatttctacttgttctttttctaaaatcaaactagtatgcatttcaacaacctggctttctaattctgatattctcaaggttaatgctgatatatctgaccccaactcatcttctcttagttgatttaaattctgaatatttgttctttcaggttctgatgaaattgtttgattatcttgacagaattttgcatattcctgaactgcctcaagttggatttgactgacaagagcagcagccactttttcttcaactattttctgtaggtttacaatcttcttttgaagcatttctgtttcaaactggccttgttcttgcatgtcttttatttgtttataacactgggtaagttctaagtcctttgcactaacagtgctctcaagttgtagcaaccttgtttccaaattaattatggaacctttgccattttcttcaaaagatttgaagtatgtctgattttctagggatttaagagcatcctctgtaaggactacttctagttcaggtttgtctttgctcagatgatctatagccacgttaacactattctctggtatgctttgaatcttttccacactttcacgttctctctttaagctgaataattcctgtgttagctgattcattttaaaattggtttctttaagtacatttttcatgaaggtcatttcttcattagcggtttctacttgctgttccaaggccagcttttcagctataaccacatccaattgatgttttaaactgtctgcttcttctgagagggaatgagcattcattgatgtcttctgtccaatatttgccaattcctgttgaagtttttcaatcacttcattgagctgctctatttcttcttctctatttctcttcacacattcttgatcactcatcaaacattctatttgggtttcaagatcccttatcagttcatttttttcttcaataaccttgttatctgttgtaattttaagttgctgctggagtttcgtaacttgttcatttaattggtcaatttctacctctttttcctgtattatttgagcaaatttcccaaatagcacatgttggtcttgagtagacatggcatcagattcctttatggcaagtcccagtttctccatgtcatccttaaataatttgttttcctgttcaagttcttgtaggcgggtagtagattcctttttctgtatttctaattgcatatgtaattgttgaacttcttcattcttattttccagttcttctctaaactgttctaattgctcttctaagtttgtaatctctttttcctttctgtctatggcatctcgttcagcctgcaattgtacttctagggacaattctggtttagcttctacagctccaaagtgttttcggtcctctaccttttgaaaagtatctgcactcacaagaagcgcctgctccagttctcttactctgaactccagtttctctatttcttcattcctttcttgtatatccctttgaagctgctctttagagagcaaaagctcactgcatttgtctgttttttctttcagatgatttgctaactgttcaacctctctagtttgatgttcactgataggctggaatcgaggaacaaccttaagttgctgttctagtttctgtatttcctgttggaatacatctctctcatgttctctgtcaatggcttgctcatctaaaaattttctcattttttctaactgcttttccaatgcttggttttgctgtcttaaatccattagttcagtatttttttcttgttccagctctataaacctactgacttgttcttccacatctatttctagagctttcacttgtttttgaaggtcatcacgtactttttcagcttgacattgtacttctagtttttccttcattaatttttctgtctcctgtagtaattgttgttcaactgggcctgcctctgctttcatagcttccttttgtctggacagtaattctctttcttcttggatctgctgttgctctgcctccaattcttgcaacctgttacttgcacataacaactcctgctcaagacgatctattatatcagttttttcctgaatttgcctttcaaaaagagttttttcatctgcatagccatcaatgacgccctcagccttactgagctccacagctagctgttctctggccctggactcctcatgaaggcgctctcgaagttcctcttggcacttaagggactctgttgcttcttgtttctgtctaaatgactcacgcatcaactctgtctgtgtcactttcgcatgttcaagctgactgctagtttcacttatggcttctaggagtttttcaactgctgcttgtagtcgagagctaatgttcagcataagttcttcattttcagggtctatttcagttccagcaaaaccactcctcacaagtcgttgtgacagctctgttccttcctcagttacttttgaccacatgttaatgtcatttcttggcatatcacttccagaataagagggaatggattcatctgtaactcttgtatgttcctcatggacacatgactttacagatgcctctgcttctgacctccaaattaggctggcagatgactggcttttactagatctatctagaatcccaaggacatggcgaccaattgtttcttcaacagctgctgttgtctttacaacttctaagaggatcttcaaaagtctattattagctttctggagtgcatacctttcattagacaaaatctcaggaggcacatcttcaggttttctgtctaattccttttctttaaatgtttgttcttcaacttctccttggttttcatttccattctgggctaattgtctattaagtctcttaatctcttcttgtagctgttcctggtcttctcgctgtctctccatttgccgcatatgtgcttgccttaacaattccgttgcctgttgatgttcttggtattgtcgtacaagttcctgtctcatatcttccaactgttcttcattcaacattagttgtctagaagcatccatgcttgacactgaaatctcatcatgaatagactgtctaactataaatgttttatctttggagaacatttcttctgaaatagtcagcacacagtcctttgattctggtatatcatggggatcactatttgataataaaatttcctttccatgttctcctaactctttactaagtggtttaaattcttctttaaatttcacatccactgtctcaaaagtctgaaaaccaatttgatcctgtgataatttcatttcattaaaataatgttgttcttgctgacacacagcatgtgcttgctttgatgatgcagtattttcttttcccccagatattctagacagttcagtttgttgagcaaatgctatactcattgacacaataaccttagctacttcttcttctaattgttcttggtattgtttttcaagcaacttaacgatatttgtttcctctttcactccaaattcaccagaaaactctattgtaccatcaatattctttttcacacaacttccagggtacattgttctctgtgcatcagattctgtaattaccaccgaatcaacaggtaagcttggcggaaccgtggactcactaacagcttgaagcctcttctgtaaacagtggatctctgcctcatagttttgttcagtttctttcaactgttgctgcaaagaggatatgaggctttctaattcttgaacttgttcttcaagtttagttttttcaagatcttgcagagaagataacttgcttttatgattgacatcaatgtcttccaaattggtcatctgagaatggattgataaaaactctgtttcctcttttggaaggttttcttctccaaattcaagtttcataccatctgtctgctgtccccagatcttgcttagtcgtgtttgaagtaccaagagtttgttgtattcttctgttactttgttgagaagagtgtgcatattttcttgaaagtcttgaacttcatatctataatcttgtaattctggatcttcattttcagaaatgtaatcaccagaattctctttgtcttctgcatttacttcacattttaaagcaggagtataatattcaccaaggacactgcataaagtctgtaaaaaataagaacattcttcagacactgccttttgaagttttccaatgagcagatgtaaaggctttccttcatcacctgtttcttgtgttttcatagtctgtagttctaactggtgtattttctgaagttccttgatcttttcctcttgagcaaaaataagctcttctttaagactgcaaagagctttatctttttcattttccatatattcacgaacctgatccacatgagttgaataaaccagagagaggcaaatgcgttgggcttccatctgtagccttaaatcattctgttctgatttaagtacattgagttctttctgaagtttatcattttcacttggttgagttgctctaagtgatgattcctttgttacagatggtaagtgatccaaaatcaactgttcttgcttactttcttctccaacagtcatattttcaaaagaaactttatcttccaccattatttttgattcttcaccaaaacttttatttactttagaaactgatccttcagcacccctgcttgtcatggtcacaactccatctaataaagagcttacttgagtatcacatgactgtacattttctgccctgttgtggttaataatgatttctagctctctacatctcaatgaaacttgttctttctcttgctttaaagatttaacttcttcatttagaaaactaatctcaccatgtttctgtttcaattgttcagaaagatcagacagtctctgtgacagctctaatttctctcgcttggttacctcaagtttttccatgagttctgttgtatccttttcaacaacctcacccatttccaatgtttctgctacaaaagttttgtcttcatcaaagacagaacttttcattttcactgtagttggatttattctttgcaaatgaagctcttcattaagtgctttaagtttacttttatactctaattcctgtttatttttactgtcttctaaatcatcttttactttgagaaggcaagcatactcctcttgtaactcttgatagttaacttcaaagtttttttcagcaaatgaaaaagtgttcctttgcttttcaatctcttcatttagctgaatacattgttgtttgaggtcctcattttcctctataagtatttctatttctttttcccacacagagtctttggatttggacttaatggagtctaagaaaatcaatctttcttcttggctaacaggagtatgtattttcaacatgtcttcaagggttttcttttcatctttaagaatgctattctctgcttcaagttgtgcaaatttttcttgaagatcattctctttttccttcatctgtttttctaacaattctgttttaagttgtaattcttgaacttcttgttcaagtgtacccttttctttttcttcttgtctgagtatttcaatttctttttgaagttcattgatttgaagagtcatttcttctgactttgaatttacaagagactgctgtaaatcttttagctttgaaatttccaaaattaattgattctgcttagttatcaaattgtccttttcaaactgcatggtttctatcttttgactcatttcattctgtaaaccatctatctgctgtttatagtgaatgcctaaattatctttaagtttttcaatatttattcgatgttcaatttctaaatcttccttcagtttggaaagctcttcttcgtgactaaatagaagctgtgttctcagcctctctaattcagcttcttgtgattcagccattctgtctaacacagcattcttttctttttctaacatttcaagttttatcttgtaatttgtaacttctgcttcatgttttaattctagttcctttctggattcagatgcagaaacaatctcagctttcaaatcttccactgtactaagggacttatgtgcttcattaagtttactttcttgttcagctattgtctgtctagctctctgaatctgttcccttgaaaagctcaattcttcaacaaggtcttcaagctgtctctgtagagcacacttttcttctaaaattagtcctagttcttccttgagtttttccttttgagagttagtatcttgcaattttatattcagttcatttattgccacattcattaactttatctgatcttcattaactgtaatatttgaatatgaccttaaagcattctccatttctcccttatgccgtgttttcatttcctccatctgtgccatgtgttgtcttattaattcttgtttcatttgcactatctgctgcccatacatctcatccagctctgcccggagttgttctaactttctttgtgtttcttgttccattcgttgtactatatcagtttcgaactggctgtctttatgatttctcttctgaagttcttcgactgtccccattaactgttttatttcttcagaagactgtctttctttttgcttagaattagtcagctctaatttcatgttttttatttcttggttcttttgcacaatctgttcttgtaattctcctagtaatttatcagcagttgttaatttatcctttagctcaagagttttcttttcttcttctattatttttgtgtttaattcttcaatgattgtctccttttcctgtatttcttctttatttgagttttctacttttttatcttgttccatttcatatactttaattttctcttgcaagaaactaatttgcattgtgaagtcttctttctttttctgataatcttctaataagtggtcttgttcttcaagctgctgttgatgagtgaggatctgttgtttggcttgtagtaagtctgcagctgtgctactatgagtgctgtttctcagagtttcactagcctgtaattgctgaaattgaatctgtaatttttgactctgttctgtcaactctaaaaattctctcattgtctcatccttttctcttcttgcttgttgtaaattagcagtgagctgggttataatgccatctctttgtttaatggcagcttcaaattcttgtaactgctgcagtccttcagtcccataggtaaccctcatttcttccagctctctgtttagctcttcaatctcatgctgcttcccagccaactcactttccatcatctctagatgagtcggactgtcttgtgctccttgttcagaataagaatcatcaacaccaaattcttcttcccttaataaatttgtaggctttcctgttctcatcacaaaactgcaaccatttacctctgaactgcagtcatctgctgtggttgaaatttcactttccagttccacagagaagccctgctcatgactggttatttctccactatgtagagttctcattattgtagattcaggaatcacagttgattctactctctgagaactatttatgtacatttcattacactgtgattgatcaatattcaaatcatggtgtgctgacacatcatgtttactgcttgacgtttttctcttttttttctgcttcttggaaggactctgcccatccgactgagcttttctttgtcgaaactgggcaagcttggctttgccggcctccagcttcttctgtctctcctcgtcctccatggcctctgcaaggaaggcaggggaaaacaggggttgaggggtggttggggatagaaaggaaaggtcgatttggacggaggtgggacggcaagctccacggcctagagagccgattcggtccggcgctcccccgcccgaagtggaagcagtctccgcgctcactggcggatcgtcctcagccgcacgggaagcgccgtcaccgccgccgccgccgccatcttcgtctccacgta

SEQ ID NO: 14226 - RNA, 12883 nt, Homo sapiens
  source 1..12883: mol_type = other RNA
gctgggattacaggcatgagccaccgcgcccagcccatatacttaagctgacttttaagagattttgaatatatatgtaaaaatcaccatgactggctctatggcaaggtaggtgagactaatatttagagtttttttaaagtgctctcaaagttggatgttctatacctcatacatttttgaaaaatcttttggtcttcaaaatctgggtcttgtgaaatttggatgctcaaaacaaaacaagcctaggcaaaccaacaaactcagctatgataataaaagtttcctattactacaagatgcttgggtgtaaacaaatgatttcttgaaggaagagataaactactcaatgattcaaagtctctgaatcaggagtgaactgaagtgagatagggaaaagaggttttccttccatgaacagggaatccacctttattttaaagtatgacttgttttttgtttttgaacaaagaaaaaataatccttacaaagtattttaaatgggatagtttttttcgatgatacataaaagcacaatatagtagcagggataatggttacattaagtgcttaaagtaagtgcttcctccttaactccacccgatttgcatgccttaccactttcttttttttttttttttctttgagacagggtctcgctctgctgcccaggctggagtgctgcggcacggccttaccactttctgccatgcgctacttaggaatacgttctccagttaggctctgtagactcagagtaccttgcacactggtgctcattgtgcattttgtgtcatcagtccgctgaatgaacatagtaggaaatcatttttgggaggagtgggatctggggtgataaatcatattttcacttaaattatttaaagtcagtttctctgctggttacaagagtttaagctttggctaacttaataattagctcatgcactaaactggaagctttgattatcctaatgagtgtgaaagaatttcaaagaaaggggagctgtgggtctcgcactgtggtgctgccaagatgtggttaaactcagagcacctgactgtatagttccaagtcgtctttgcagtgcctctagccgagtgatataatctgttagggctctgtcaggatcgtaattctgaagctgagaacatgctaaagaaccaggattgaaatcagctggagtgcctgggtacctattctgaaatggtaaaggggacctaatatagtccagatctgatcttgagcgatacgtagtatgtcttggttctccatataactccagcccaccagaagaatgataaaatgagtcagtcttttctgcaccttgattcagtccaaagccatctctgttaatattgatggaaacagaacctgtgactcgatgccaccgtcgaaccaaaaatttcattctggaaattgcaatggatactctgacggccgaccgaaacctggtgaagccctttgggcgattggtgatcacctctagatccgtgaaagctggctgcccccccatccgggcaagcagggccaaggtggcatcttcacattcctggaacccacccagtaacagcagcaggtatttcttctggtaaatgagagcctttcgaaaactttctgccctcaagtatttaccataaattctctttaaagtgacatgttcagaatcagggctcagagtttgaagtaaagagtcatttcttagttcagctttcagtttgtatacttcagcctctgcccttttcaaagatttctggagagtcaatttttctctgttccatacttctttttcagaggcaatgatggcttcaatgttggcaccaccattcaatgaaaacctggaagaattatctctaccagctcctgtctgtcgataccacctgatctgctcttccagcttcataaccatgttccttaagtcattcttctcttcagtcagttgactgatatgccctgtcagctcagcattttgtctcagtagtctttcagtcaatgagccacaagaagtacttggggacaccaagctgggctcttcaccttgctggccagttaatttctgtagttgtaaaataatttcatcaatattttcctgaacccaaatgaaatcttcatcatctgctgtttcaaactgtagtctctcagaggctttctggggtagaacctgtagttttgaagctacacattgaagcttttgtctgatcatttctaattcatgattacagccggttcctcctccattcatttcaatcaatttagcgtagtttgattcttttgtttctccttctattttctgttgaagaacccaatttctagttctatcactggttaagctccacgtggttggctcattaaggttctgatacagaattcttctactttctcgtttttcttctcgttctagttcttgcttctggaattcctgcatgattccttgtagtcgctgtccttcaaggtctaacttataaacttgttgtcttttctcttccagctggcgctgaagatcttccactttggactggagctcatgcatttttttctgtccctcagtgttggcctcctgttctgtctgcagtgttttcctgtgaacctgcctatctttttccatttgctgtcgtgtttgcaaagaatccagtttatatttttcagtctcatttaacaattctactatgcgactgtgtttttcctctagctgtttctgcagctctttcagtaggtcctctgagggcaagggtggccgagactgtccagtaccatcactgctctgcagctgtgcgtgcaattcccgctccctatctagggtactactcatttcccgaattcgaactttctcagattcaagaagtacctgaagctctaagtttcgaccttgttcttctgacaactgggcatcatatagcattctctgtgattctattttttgctgggattcgttcagtagttgtttctgttgttccaaaagtagatttagctgaagattcctttgtttctgactctcaagtgaaaacttcagatcctcaagttcttctttatcccgttcttcactgcgtcccaacttggctttctctttctccaaagcccactggagctctcttgattttttctgttcacttgctaatgtgtcattaagcaaatgtacttcatctgtcttatctttaacttccaacctgaaagcctccaattcttttaggtgtttatgctgtgccttgagtgttgtttctagttccaatttagtttgtgcaagctcactcttcagttcagcaaccaccattttctcagaactcagctgctcctgcagttccgttgctctgtctttcatactgctgagctccacttgcatctccagcatttgagactgcttctgctgtatattatattccaagagttcttggcttggtttctcactctcttgttctcttttcagagtaattttcctaccattcatttgtgcatgcagtgcctgaatttcagataacaaactccttctatctgctttctggaggcattccatagctgcttgatattcaacaccctgttcttgtattctctgttccaaacagtttagtaaaccaactgcatctgtagtacctagagctgtcagctccgtccgaaatgctgctagtaaaacactacgctcttctaagaaaacttgttgaagggcaagcagtagttcacctcgccagtctgagaagctctcatgagattgagaactatcataaacctcggcttctctttgcagttgcatctttgtaattaaatcctttagagatgagattgtattgatgtaagcttttctctcttctagccaaggttctgaaacctgctgaatagaatggtcctctccatcactatagggagactcagtgagagaaagcacctgcatgccttcattatggacagctctcagtaatccctttattttctttggaaaggaatctgttgcactttcactttcttctcctcggccttctgatgctatgtcaaatccctgactgtgtgtaagataaattccctgaccccagtctgatccagaatcactggagcatatttctctagtctggtaagcatcagaatgtgctagctcaggaattgaggatccctctttacttctcagacactgtatcactgccttcaaggtaccacattcctctttcagtaactgaacggcaacatagtgttccctctttaaggtttcagtttctgaaatatgtctggattccatgtccaaaatttcagcagcatgtagttcttgcatcttctcaattttttcagtaaactgactgattatttcagtaacttcttctgaggaacattcactctgtaaattaatttgtattcctgcatttttaacaagaatttgtggagtctgattgctgctactgatcttcagagtcccatctgtctgggatgcaatgctcttactcagttttataggaagtggctcaaacatgcaggcctttttgctttcttgtacctcagtctcatcttctttttctaaaatggacaatttctcttttgcctctgcgaggtgatccctaacttggcttaagtctttctgaagagatgtcatatttgtttcttttaccaaaagctcttcttgaagtttttcagccttttctttataactggcaagttctgctttggtagccactgattcagctctaagagcctcgagttcattaaaaaatccactttcttcattgctatgaaatagctcagtagttgtcttgagaacttcaacatcttgagggcttcttttcttttctttctctctctgttttttctcattgccctccaatagcttctgtagttctagcagcttcttttctttttctaaaacatttttttctgcaatttctacttgttctttttctaaaatcaaactagtatgcatttcaacaacctggctttctaattctgatattctcaaggttaatgctgatatatctgaccccaactcatcttctcttagttgatttaaattctgaatatttgttctttcaggttctgatgaaattgtttgattatcttgacagaattttgcatattcctgaactgcctcaagttggatttgactgacaagagcagcagccactttttcttcaactattttctgtaggtttacaatcttcttttgaagcatttctgtttcaaactggccttgttcttgcatgtcttttatttgtttataacactgggtaagttctaagtcctttgcactaacagtgctctcaagttgtagcaaccttgtttccaaattaattatggaacctttgccattttcttcaaaagatttgaagtatgtctgattttctagggatttaagagcatcctctgtaaggactacttctagttcaggtttgtctttgctcagatgatctatagccacgttaacactattctctggtatgctttgaatcttttccacactttcacgttctctctttaagctgaataattcctgtgttagctgattcattttaaaattggtttctttaagtacatttttcatgaaggtcatttcttcattagcggtttctacttgctgttccaaggccagcttttcagctataaccacatccaattgatgttttaaactgtctgcttcttctgagagggaatgagcattcattgatgtcttctgtccaatatttgccaattcctgttgaagtttttcaatcacttcattgagctgctctatttcttcttctctatttctcttcacacattcttgatcactcatcaaacattctatttgggtttcaagatcccttatcagttcatttttttcttcaataaccttgttatctgttgtaattttaagttgctgctggagtttcgtaacttgttcatttaattggtcaatttctacctctttttcctgtattatttgagcaaatttcccaaatagcacatgttggtcttgagtagacatggcatcagattcctttatggcaagtcccagtttctccatgtcatccttaaataatttgttttcctgttcaagttcttgtaggcgggtagtagattcctttttctgtatttctaattgcatatgtaattgttgaacttcttcattcttattttccagttcttctctaaactgttctaattgctcttctaagtttgtaatctctttttcctttctgtctatggcatctcgttcagcctgcaattgtacttctagggacaattctggtttagcttctacagctccaaagtgttttcggtcctctaccttttgaaaagtatctgcactcacaagaagcgcctgctccagttctcttactctgaactccagtttctctatttcttcattcctttcttgtatatccctttgaagctgctctttagagagcaaaagctcactgcatttgtctgttttttctttcagatgatttgctaactgttcaacctctctagtttgatgttcactgataggctggaatcgaggaacaaccttaagttgctgttctagtttctgtatttcctgttggaatacatctctctcatgttctctgtcaatggcttgctcatctaaaaattttctcattttttctaactgcttttccaatgcttggttttgctgtcttaaatccattagttcagtatttttttcttgttccagctctataaacctactgacttgttcttccacatctatttctagagctttcacttgtttttgaaggtcatcacgtactttttcagcttgacattgtacttctagtttttccttcattaatttttctgtctcctgtagtaattgttgttcaactgggcctgcctctgctttcatagcttccttttgtctggacagtaattctctttcttcttggatctgctgttgctctgcctccaattcttgcaacctgttacttgcacataacaactcctgctcaagacgatctattatatcagttttttcctgaatttgcctttcaaaaagagttttttcatctgcatagccatcaatgacgccctcagccttactgagctccacagctagctgttctctggccctggactcctcatgaaggcgctctcgaagttcctcttggcacttaagggactctgttgcttcttgtttctgtctaaatgactcacgcatcaactctgtctgtgtcactttcgcatgttcaagctgactgctagtttcacttatggcttctaggagtttttcaactgctgcttgtagtcgagagctaatgttcagcataagttcttcattttcagggtctatttcagttccagcaaaaccactcctcacaagtcgttgtgacagctctgttccttcctcagttacttttgaccacatgttaatgtcatttcttggcatatcacttccagaataagagggaatggattcatctgtaactcttgtatgttcctcatggacacatgactttacagatgcctctgcttctgacctccaaattaggctggcagatgactggcttttactagatctatctagaatcccaaggacatggcgaccaattgtttcttcaacagctgctgttgtctttacaacttctaagaggatcttcaaaagtctattattagctttctggagtgcatacctttcattagacaaaatctcaggaggcacatcttcaggttttctgtctaattccttttctttaaatgtttgttcttcaacttctccttggttttcatttccattctgtgtttgcgtactgctgttgcgcagctcacaacacagcttctctcttccagctaaagacagctgctttagtgcttccagctcctctaaaagcaccctctctctctctgaaaccaggttttcattatctatggaggatctctgggctaattgtctattaagtctcttaatctcttcttgtagctgttcctggtcttctcgctgtctctccatttgccgcatatgtgcttgccttaacaattccgttgcctgttgatgttcttggtattgtcgtacaagttcctgtctcatatcttccaactgttcttcattcaacattagttgtctagaagcatccatgcttgacactgaaatctcatcatgaatagactgtctaactataaatgttttatctttggagaacatttcttctgaaatagtcagcacacagtcctttgattctggtatatcatggggatcactatttgataataaaatttcctttccatgttctcctaactctttactaagtggtttaaattcttctttaaatttcacatccactgtctcaaaagtctgaaaaccaatttgatcctgtgataatttcatttcattaaaataatgttgttcttgctgacacacagcatgtgcttgctttgatgatgcagtattttcttttcccccagatattctagacagttcagtttgttgagcaaatgctatactcattgacacaataacctctattgtaccatcaatattctttttcacacaacttccagggtacattgttctctgtgcatcagattctgtaattaccaccgaatcaacaggtaagcttggcggaaccgtggactcactaacagcttgaagcctcttctgtaaacagtggatctctgcctcatagttttgttcagtttctttcaactgttgctgcaaagaggatatgaggctttctaattcttgaacttgttcttcaagtttagttttttcaagatcttgcagagaagataacttgcttttatgattgacatcaatgtcttccaaattggtcatctgagaatggattgataaaaactctgtttcctcttttggaaggttttcttctccaaattcaagtttcataccatctgtctgctgtccccagatcttgcttagtcgtgtttgaagtaccaagagtttgttgtattcttctgttactttgttgagaagagtgtgcatattttcttgaaagtcttgaacttcatatctataatcttgtaattctggatcttcattttcagaaatgtaatcaccagaattctctttgtcttctgcatttacttcacattttaaagcaggagtataatattcaccaaggacactgcataaagtctgtaaaaaataagaacattcttcagacactgccttttgaagttttccaatgagcagatgtaaaggctttccttcatcacctgtttcttgtgttttcatagtctgtagttctaactggtgtattttctgaagttccttgatcttttcctcttgagcaaaaataagctcttctttaagactgcaaagagctttatctttttcattttccatatattcacgaacctgatccacatgagttgaataaaccagagagaggcaaatgcgttgggcttccatctgtagccttaaatcattctgttctgatttaagtacattgagttctttctgaagtttatcattttcacttggttgagttgctctaagtgatgattcctttgttacagatggtaagtgatccaaaatcaactgttcttgcttactttcttctccaacagtcatattttcaaaagaaactttatcttccaccattatttttgattcttcaccaaaacttttatttactttagaaactgatccttcagcacccctgcttgtcatggtcacaactccatctaataaagagcttacttgagtatcacatgactgtacattttctgccctgttgtggttaataatgatttctagctctctacatctcaatgaaacttgttctttctcttgctttaaagatttaacttcttcatttagaaaactaatctcaccatgtttctgtttcaattgttcagaaagatcagacagtctctgtgacagctctaatttctctcgcttggttacctcaagtttttccatgagttctgttgtatccttttcaacaacctcacccatttccaatgtttctgctacaaaagttttgtcttcatcaaagacagaacttttcattttcactgtagttggatttattctttgcaaatgaagctcttcattaagtgctttaagtttacttttatactctaattcctgtttatttttactgtcttctaaatcatcttttactttgagaaggcaagcatactcctcttgtaactcttgatagttaacttcaaagtttttttcagcaaatgaaaaagtgttcctttgcttttcaatctcttcatttagctgaatacattgttgtttgaggtcctcattttcctctataagtatttctatttctttttcccacacagagtctttggatttggacttaatggagtctaagaaaatcaatctttcttcttggctaacaggagtatgtattttcaacatgtcttcaagggttttcttttcatctttaagaatgctattctctgcttcaagttgtgcaaatttttcttgaagatcattctctttttccttcatctgtttttctaacaattctgttttaagttgtaattcttgaacttcttgttcaagtgtacccttttctttttcttcttgtctgagtatttcaatttctttttgaagttcattgatttgaagagtcatttcttctgactttgaatttacaagagactgctgtaaatcttttagctttgaaatttccaaaattaattgattctgcttagttatcaaattgtccttttcaaactgcatggtttctatcttttgactcatttcattctgtaaaccatctatctgctgtttatagtgaatgcctaaattatctttaagtttttcaatatttattcgatgttcaatttctaaatcttccttcagtttggaaagctcttcttcgtgactaaatagaagctgtgttctcagcctctctaattcagcttcttgtgattcagccattctgtctaacacagcattcttttctttttctaacatttcaagttttatcttgtaatttgtaacttctgcttcatgttttaattctagttcctttctggattcagatgcagaaacaatctcagctttcaaatcttccactgtactaagggacttatgtgcttcattaagtttactttcttgttcagctattgtctgtctagctctctgaatctgttcccttgaaaagctcaattcttcaacaaggtcttcaagctgtctctgtagagcacacttttcttctaaaattagtcctagttcttccttgagtttttccttttgagagttagtatcttgcaattttatattcagttcatttattgccacattcattaactttatctgatcttcattaactgtaatatttgaatatgaccttaaagcattctccatttctcccttatgccgtgttttcatttcctccatctgtgccatgtgttgtcttattaattcttgtttcatttgcactatctgctgcccatacatctcatccagctctgcccggagttgttctaactttctttgtgtttcttgttccattcgttgtactatatcagtttcgaactggctgtctttatgatttctcttctgaagttcttcgactgtccccattaactgttttatttcttcagaagactgtctttctttttgcttagaattagtcagctctaatttcatgttttttatttcttggttcttttgcacaatctgttcttgtaattctcctagtaatttatcagcagttgttaatttatcctttagctcaagagttttcttttcttcttctattatttttgtgtttaattcttcaatgattgtctccttttcctgtatttcttctttatttgagttttctacttttttatcttgttccatttcatatactttaattttctcttgcaagaaactaatttgcattgtgaagtcttctttctttttctgataatcttctaataagtggtcttgttcttcaagctgctgttgatgagtgaggatctgttgtttggcttgtagtaagtctgcagctgtgctactatgagtgctgtttctcagagtttcactagcctgtaattgctgaaattgaatctgtaatttttgactctgttctgtcaactctaaaaattctctcattgtctcatccttttctcttcttgcttgttgtaaattagcagtgagctgggttataatgccatctctttgtttaatggcagcttcaaattcttgtaactgctgcagtccttcagtcccataggtaaccctcatttcttccagctctctgtttagctcttcaatctcatgctgcttcccagccaactcactttccatcatctctagatgagtcggactgtcttgtgctccttgttcagaataagaatcatcaacaccaaattcttcttcccttaataaatttgtaggctttcctgttctcatcacaaaactgcaaccatttacctctgaactgcagtcatctgctgtggttgaaatttcactttccagttccacagagaagccctgctcatgactggttatttctccactatgtagagttctcattattgtagattcaggaatcacagttgattctactctctgagaactatttatgtacatttcattacactgtgattgatcaatattcaaatcatggtgtgctgacacatcatgtttactgcttgacgtttttctcttttttttctgcttcttggaaggactctgcccatccgactgagcttttctttgtcgaaactgggcaagcttggctttgccggcctccagcttcttctgtctctcctcgtcctccatggcctctgcaaggaaggcaggggaaaacaggggttgaggggtggttggggatagaaaggaaaggtcgatttggacggaggtgggacggcaagctccacggcctagagagccgattcggtccggcgctcccccgcccgaagtggaagcagtctccgcgctcactggcggatcgtcctcagccgcacgggaagcgccgtcaccgccgccgccgccgccatcttcgtctccacgta

SEQ ID NO: 14227 - RNA, 12976 nt, Homo sapiens
  source 1..12976: mol_type = other RNA
gctgggattacaggcatgagccaccgcgcccagcccatatacttaagctgacttttaagagattttgaatatatatgtaaaaatcaccatgactggctctatggcaaggtaggtgagactaatatttagagtttttttaaagtgctctcaaagttggatgttctatacctcatacatttttgaaaaatcttttggtcttcaaaatctgggtcttgtgaaatttggatgctcaaaacaaaacaagcctaggcaaaccaacaaactcagctatgataataaaagtttcctattactacaagatgcttgggtgtaaacaaatgatttcttgaaggaagagataaactactcaatgattcaaagtctctgaatcaggagtgaactgaagtgagatagggaaaagaggttttccttccatgaacagggaatccacctttattttaaagtatgacttgttttttgtttttgaacaaagaaaaaataatccttacaaagtattttaaatgggatagtttttttcgatgatacataaaagcacaatatagtagcagggataatggttacattaagtgcttaaagtaagtgcttcctccttaactccacccgatttgcatgccttaccactttcttttttttttttttttctttgagacagggtctcgctctgctgcccaggctggagtgctgcggcacggccttaccactttctgccatgcgctacttaggaatacgttctccagttaggctctgtagactcagagtaccttgcacactggtgctcattgtgcattttgtgtcatcagtccgctgaatgaacatagtaggaaatcatttttgggaggagtgggatctggggtgataaatcatattttcacttaaattatttaaagtcagtttctctgctggttacaagagtttaagctttggctaacttaataattagctcatgcactaaactggaagctttgattatcctaatgagtgtgaaagaatttcaaagaaaggggagctgtgggtctcgcactgtggtgctgccaagatgtggttaaactcagagcacctgactgtatagttccaagtcgtctttgcagtgcctctagccgagtgatataatctgttagggctctgtcaggatcgtaattctgaagctgagaacatgctaaagaaccaggattgaaatcagctggagtgcctgggtacctattctgaaatggtaaaggggacctaatatagtccagatctgatcttgagcgatacgtagtatgtcttggttctccatataactccagcccaccagaagaatgataaaatgagtcagtcttttctgcaccttgattcagtccaaagccatctctgttaatattgatggaaacagaacctgtgactcgatgccaccgtcgaaccaaaaatttcattctggaaattgcaatggatactctgacggccgaccgaaacctggtgaagccctttgggcgattggtgatcacctctagatccgtgaaagctggctgcccccccatccgggcaagcagggccaaggtggcatcttcacattcctggaacccacccagtaacagcagcaggtatttcttctggtaaatgagagcctttcgaaaactttctgccctcaagtatttaccataaattctctttaaagtgacatgttcagaatcagggctcagagtttgaagtaaagagtcatttcttagttcagctttcagtttgtatacttcagcctctgcccttttcaaagatttctggagagtcaatttttctctgttccatacttctttttcagaggcaatgatggcttcaatgttggcaccaccattcaatgaaaacctggaagaattatctctaccagctcctgtctgtcgataccacctgatctgctcttccagcttcataaccatgttccttaagtcattcttctcttcagtcagttgactgatatgccctgtcagctcagcattttgtctcagtagtctttcagtcaatgagccacaagaagtacttggggacaccaagctgggctcttcaccttgctggccagttaatttctgtagttgtaaaataatttcatcaatattttcctgaacccaaatgaaatcttcatcatctgctgtttcaaactgtagtctctcagaggctttctggggtagaacctgtagttttgaagctacacattgaagcttttgtctgatcatttctaattcatgattacagccggttcctcctccattcatttcaatcaatttagcgtagtttgattcttttgtttctccttctattttctgttgaagaacccaatttctagttctatcactggttaagctccacgtggttggctcattaaggttctgatacagaattcttctactttctcgtttttcttctcgttctagttcttgcttctggaattcctgcatgattccttgtagtcgctgtccttcaaggtctaacttataaacttgttgtcttttctcttccagctggcgctgaagatcttccactttggactggagctcatgcatttttttctgtccctcagtgttggcctcctgttctgtctgcagtgttttcctgtgaacctgcctatctttttccatttgctgtcgtgtttgcaaagaatccagtttatatttttcagtctcatttaacaattctactatgcgactgtgtttttcctctagctgtttctgcagctctttcagtaggtcctctgagggcaagggtggccgagactgtccagtaccatcactgctctgcagctgtgcgtgcaattcccgctccctatctagggtactactcatttcccgaattcgaactttctcagattcaagaagtacctgaagctctaagtttcgaccttgttcttctgacaactgggcatcatatagcattctctgtgattctattttttgctgggattcgttcagtagttgtttctgttgttccaaaagtagatttagctgaagattcctttgtttctgactctcaagtgaaaacttcagatcctcaagttcttctttatcccgttcttcactgcgtcccaacttggctttctctttctccaaagcccactggagctctcttgattttttctgttcacttgctaatgtgtcattaagcaaatgtacttcatctgtcttatctttaacttccaacctgaaagcctccaattcttttaggtgtttatgctgtgccttgagtgttgtttctagttccaatttagtttgtgcaagctcactcttcagttcagcaaccaccattttctcagaactcagctgctcctgcagttccgttgctctgtctttcatactgctgagctccacttgcatctccagcatttgagactgcttctgctgtatattatattccaagagttcttggcttggtttctcactctcttgttctcttttcagagtaattttcctaccattcatttgtgcatgcagtgcctgaatttcagataacaaactccttctatctgctttctggaggcattccatagctgcttgatattcaacaccctgttcttgtattctctgttccaaacagtttagtaaaccaactgcatctgtagtacctagagctgtcagctccgtccgaaatgctgctagtaaaacactacgctcttctaagaaaacttgttgaagggcaagcagtagttcacctcgccagtctgagaagctctcatgagattgagaactatcataaacctcggcttctctttgcagttgcatctttgtaattaaatcctttagagatgagattgtattgatgtaagcttttctctcttctagccaaggttctgaaacctgctgaatagaatggtcctctccatcactatagggagactcagtgagagaaagcacctgcatgccttcattatggacagctctcagtaatccctttattttctttggaaaggaatctgttgcactttcactttcttctcctcggccttctgatgctatgtcaaatccctgactgtgtgtaagataaattccctgaccccagtctgatccagaatcactggagcatatttctctagtctggtaagcatcagaatgtgctagctcaggaattgaggatccctctttacttctcagacactgtatcactgccttcaaggtaccacattcctctttcagtaactgaacggcaacatagtgttccctctttaaggtttcagtttctgaaatatgtctggattccatgtccaaaatttcagcagcatgtagttcttgcatcttctcaattttttcagtaaactgactgattatttcagtaacttcttctgaggaacattcactctgtaaattaatttgtattcctgcatttttaacaagaatttgtggagtctgattgctgctactgatcttcagagtcccatctgtctgggatgcaatgctcttactcagttttataggaagtggctcaaacatgcaggcctttttgctttcttgtacctcagtctcatcttctttttctaaaatggacaatttctcttttgcctctgcgaggtgatccctaacttggcttaagtctttctgaagagatgtcatatttgtttcttttaccaaaagctcttcttgaagtttttcagccttttctttataactggcaagttctgctttggtagccactgattcagctctaagagcctcgagttcattaaaaaatccactttcttcattgctatgaaatagctcagtagttgtcttgagaacttcaacatcttgagggcttcttttcttttctttctctctctgttttttctcattgccctccaatagcttctgtagttctagcagcttcttttctttttctaaaacatttttttctgcaatttctacttgttctttttctaaaatcaaactagtatgcatttcaacaacctggctttctaattctgatattctcaaggttaatgctgatatatctgaccccaactcatcttctcttagttgatttaaattctgaatatttgttctttcaggttctgatgaaattgtttgattatcttgacagaattttgcatattcctgaactgcctcaagttggatttgactgacaagagcagcagccactttttcttcaactattttctgtaggtttacaatcttcttttgaagcatttctgtttcaaactggccttgttcttgcatgtcttttatttgtttataacactgggtaagttctaagtcctttgcactaacagtgctctcaagttgtagcaaccttgtttccaaattaattatggaacctttgccattttcttcaaaagatttgaagtatgtctgattttctagggatttaagagcatcctctgtaaggactacttctagttcaggtttgtctttgctcagatgatctatagccacgttaacactattctctggtatgctttgaatcttttccacactttcacgttctctctttaagctgaataattcctgtgttagctgattcattttaaaattggtttctttaagtacatttttcatgaaggtcatttcttcattagcggtttctacttgctgttccaaggccagcttttcagctataaccacatccaattgatgttttaaactgtctgcttcttctgagagggaatgagcattcattgatgtcttctgtccaatatttgccaattcctgttgaagtttttcaatcacttcattgagctgctctatttcttcttctctatttctcttcacacattcttgatcactcatcaaacattctatttgggtttcaagatcccttatcagttcatttttttcttcaataaccttgttatctgttgtaattttaagttgctgctggagtttcgtaacttgttcatttaattggtcaatttctacctctttttcctgtattatttgagcaaatttcccaaatagcacatgttggtcttgagtagacatggcatcagattcctttatggcaagtcccagtttctccatgtcatccttaaataatttgttttcctgttcaagttcttgtaggcgggtagtagattcctttttctgtatttctaattgcatatgtaattgttgaacttcttcattcttattttccagttcttctctaaactgttctaattgctcttctaagtttgtaatctctttttcctttctgtctatggcatctcgttcagcctgcaattgtacttctagggacaattctggtttagcttctacagctccaaagtgttttcggtcctctaccttttgaaaagtatctgcactcacaagaagcgcctgctccagttctcttactctgaactccagtttctctatttcttcattcctttcttgtatatccctttgaagctgctctttagagagcaaaagctcactgcatttgtctgttttttctttcagatgatttgctaactgttcaacctctctagtttgatgttcactgataggctggaatcgaggaacaaccttaagttgctgttctagtttctgtatttcctgttggaatacatctctctcatgttctctgtcaatggcttgctcatctaaaaattttctcattttttctaactgcttttccaatgcttggttttgctgtcttaaatccattagttcagtatttttttcttgttccagctctataaacctactgacttgttcttccacatctatttctagagctttcacttgtttttgaaggtcatcacgtactttttcagcttgacattgtacttctagtttttccttcattaatttttctgtctcctgtagtaattgttgttcaactgggcctgcctctgctttcatagcttccttttgtctggacagtaattctctttcttcttggatctgctgttgctctgcctccaattcttgcaacctgttacttgcacataacaactcctgctcaagacgatctattatatcagttttttcctgaatttgcctttcaaaaagagttttttcatctgcatagccatcaatgacgccctcagccttactgagctccacagctagctgttctctggccctggactcctcatgaaggcgctctcgaagttcctcttggcacttaagggactctgttgcttcttgtttctgtctaaatgactcacgcatcaactctgtctgtgtcactttcgcatgttcaagctgactgctagtttcacttatggcttctaggagtttttcaactgctgcttgtagtcgagagctaatgttcagcataagttcttcattttcagggtctatttcagttccagcaaaaccactcctcacaagtcgttgtgacagctctgttccttcctcagttacttttgaccacatgttaatgtcatttcttggcatatcacttccagaataagagggaatggattcatctgtaactcttgtatgttcctcatggacacatgactttacagatgcctctgcttctgacctccaaattaggctggcagatgactggcttttactagatctatctagaatcccaaggacatggcgaccaattgtttcttcaacagctgctgttgtctttacaacttctaagaggatcttcaaaagtctattattagctttctggagtgcatacctttcattagacaaaatctcaggaggcacatcttcaggttttctgtctaattccttttctttaaatgtttgttcttcaacttctccttggttttcatttccattctgtgtttgcgtactgctgttgcgcagctcacaacacagcttctctcttccagctaaagacagctgctttagtgcttccagctcctctaaaagcaccctctctctctctgaaaccaggttttcattatctatggaggatctctgggctaattgtctattaagtctcttaatctcttcttgtagctgttcctggtcttctcgctgtctctccatttgccgcatatgtgcttgccttaacaattccgttgcctgttgatgttcttggtattgtcgtacaagttcctgtctcatatcttccaactgttcttcattcaacattagttgtctagaagcatccatgcttgacactgaaatctcatcatgaatagactgtctaactataaatgttttatctttggagaacatttcttctgaaatagtcagcacacagtcctttgattctggtatatcatggggatcactatttgataataaaatttcctttccatgttctcctaactctttactaagtggtttaaattcttctttaaatttcacatccactgtctcaaaagtctgaaaaccaatttgatcctgtgataatttcatttcattaaaataatgttgttcttgctgacacacagcatgtgcttgctttgatgatgcagtattttcttttcccccagatattctagacagttcagtttgttgagcaaatgctatactcattgacacaataaccttagctacttcttcttctaattgttcttggtattgtttttcaagcaacttaacgatatttgtttcctctttcactccaaattcaccagaaaactctattgtaccatcaatattctttttcacacaacttccagggtacattgttctctgtgcatcagattctgtaattaccaccgaatcaacaggtaagcttggcggaaccgtggactcactaacagcttgaagcctcttctgtaaacagtggatctctgcctcatagttttgttcagtttctttcaactgttgctgcaaagaggatatgaggctttctaattcttgaacttgttcttcaagtttagttttttcaagatcttgcagagaagataacttgcttttatgattgacatcaatgtcttccaaattggtcatctgagaatggattgataaaaactctgtttcctcttttggaaggttttcttctccaaattcaagtttcataccatctgtctgctgtccccagatcttgcttagtcgtgtttgaagtaccaagagtttgttgtattcttctgttactttgttgagaagagtgtgcatattttcttgaaagtcttgaacttcatatctataatcttgtaattctggatcttcattttcagaaatgtaatcaccagaattctctttgtcttctgcatttacttcacattttaaagcaggagtataatattcaccaaggacactgcataaagtctgtaaaaaataagaacattcttcagacactgccttttgaagttttccaatgagcagatgtaaaggctttccttcatcacctgtttcttgtgttttcatagtctgtagttctaactggtgtattttctgaagttccttgatcttttcctcttgagcaaaaataagctcttctttaagactgcaaagagctttatctttttcattttccatatattcacgaacctgatccacatgagttgaataaaccagagagaggcaaatgcgttgggcttccatctgtagccttaaatcattctgttctgatttaagtacattgagttctttctgaagtttatcattttcacttggttgagttgctctaagtgatgattcctttgttacagatggtaagtgatccaaaatcaactgttcttgcttactttcttctccaacagtcatattttcaaaagaaactttatcttccaccattatttttgattcttcaccaaaacttttatttactttagaaactgatccttcagcacccctgcttgtcatggtcacaactccatctaataaagagcttacttgagtatcacatgactgtacattttctgccctgttgtggttaataatgatttctagctctctacatctcaatgaaacttgttctttctcttgctttaaagatttaacttcttcatttagaaaactaatctcaccatgtttctgtttcaattgttcagaaagatcagacagtctctgtgacagctctaatttctctcgcttggttacctcaagtttttccatgagttctgttgtatccttttcaacaacctcacccatttccaatgtttctgctacaaaagttttgtcttcatcaaagacagaacttttcattttcactgtagttggatttattctttgcaaatgaagctcttcattaagtgctttaagtttacttttatactctaattcctgtttatttttactgtcttctaaatcatcttttactttgagaaggcaagcatactcctcttgtaactcttgatagttaacttcaaagtttttttcagcaaatgaaaaagtgttcctttgcttttcaatctcttcatttagctgaatacattgttgtttgaggtcctcattttcctctataagtatttctatttctttttcccacacagagtctttggatttggacttaatggagtctaagaaaatcaatctttcttcttggctaacaggagtatgtattttcaacatgtcttcaagggttttcttttcatctttaagaatgctattctctgcttcaagttgtgcaaatttttcttgaagatcattctctttttccttcatctgtttttctaacaattctgttttaagttgtaattcttgaacttcttgttcaagtgtacccttttctttttcttcttgtctgagtatttcaatttctttttgaagttcattgatttgaagagtcatttcttctgactttgaatttacaagagactgctgtaaatcttttagctttgaaatttccaaaattaattgattctgcttagttatcaaattgtccttttcaaactgcatggtttctatcttttgactcatttcattctgtaaaccatctatctgctgtttatagtgaatgcctaaattatctttaagtttttcaatatttattcgatgttcaatttctaaatcttccttcagtttggaaagctcttcttcgtgactaaatagaagctgtgttctcagcctctctaattcagcttcttgtgattcagccattctgtctaacacagcattcttttctttttctaacatttcaagttttatcttgtaatttgtaacttctgcttcatgttttaattctagttcctttctggattcagatgcagaaacaatctcagctttcaaatcttccactgtactaagggacttatgtgcttcattaagtttactttcttgttcagctattgtctgtctagctctctgaatctgttcccttgaaaagctcaattcttcaacaaggtcttcaagctgtctctgtagagcacacttttcttctaaaattagtcctagttcttccttgagtttttccttttgagagttagtatcttgcaattttatattcagttcatttattgccacattcattaactttatctgatcttcattaactgtaatatttgaatatgaccttaaagcattctccatttctcccttatgccgtgttttcatttcctccatctgtgccatgtgttgtcttattaattcttgtttcatttgcactatctgctgcccatacatctcatccagctctgcccggagttgttctaactttctttgtgtttcttgttccattcgttgtactatatcagtttcgaactggctgtctttatgatttctcttctgaagttcttcgactgtccccattaactgttttatttcttcagaagactgtctttctttttgcttagaattagtcagctctaatttcatgttttttatttcttggttcttttgcacaatctgttcttgtaattctcctagtaatttatcagcagttgttaatttatcctttagctcaagagttttcttttcttcttctattatttttgtgtttaattcttcaatgattgtctccttttcctgtatttcttctttatttgagttttctacttttttatcttgttccatttcatatactttaattttctcttgcaagaaactaatttgcattgtgaagtcttctttctttttctgataatcttctaataagtggtcttgttcttcaagctgctgttgatgagtgaggatctgttgtttggcttgtagtaagtctgcagctgtgctactatgagtgctgtttctcagagtttcactagcctgtaattgctgaaattgaatctgtaatttttgactctgttctgtcaactctaaaaattctctcattgtctcatccttttctcttcttgcttgttgtaaattagcagtgagctgggttataatgccatctctttgtttaatggcagcttcaaattcttgtaactgctgcagtccttcagtcccataggtaaccctcatttcttccagctctctgtttagctcttcaatctcatgctgcttcccagccaactcactttccatcatctctagatgagtcggactgtcttgtgctccttgttcagaataagaatcatcaacaccaaattcttcttcccttaataaatttgtaggctttcctgttctcatcacaaaactgcaaccatttacctctgaactgcagtcatctgctgtggttgaaatttcactttccagttccacagagaagccctgctcatgactggttatttctccactatgtagagttctcattattgtagattcaggaatcacagttgattctactctctgagaactatttatgtacatttcattacactgtgattgatcaatattcaaatcatggtgtgctgacacatcatgtttactgcttgacgtttttctcttttttttctgcttcttggaaggactctgcccatccgactgagcttttctttgtcgaaactgggcaagcttggctttgccggcctccagcttcttctgtctctcctcgtcctccatggcctctgcaaggaaggcaggggaaaacaggggttgaggggtggttggggatagaaaggaaaggtcgatttggacggaggtgggacggcaagctccacggcctagagagccgattcggtccggcgctcccccgcccgaagtggaagcagtctccgcgctcactggcggatcgtcctcagccgcacgggaagcgccgtcaccgccgccgccgccgccatcttcgtctccacgta

SEQ ID NO: 14228 - RNA, 7943 nt, Homo sapiens
  source 1..7943: mol_type = other RNA
gctgggattacaggcatgagccaccgcgcccagcccatatacttaagctgacttttaagagattttgaatatatatgtaaaaatcaccatgactggctctatggcaaggtaggtgagactaatatttagagtttttttaaagtgctctcaaagttggatgttctatacctcatacatttttgaaaaatcttttggtcttcaaaatctgggtcttgtgaaatttggatgctcaaaacaaaacaagcctaggcaaaccaacaaactcagctatgataataaaagtttcctattactacaagatgcttgggtgtaaacaaatgatttcttgaaggaagagataaactactcaatgattcaaagtctctgaatcaggagtgaactgaagtgagatagggaaaagaggttttccttccatgaacagggaatccacctttattttaaagtatgacttgttttttgtttttgaacaaagaaaaaataatccttacaaagtattttaaatgggatagtttttttcgatgatacataaaagcacaatatagtagcagggataatggttacattaagtgcttaaagtaagtgcttcctccttaactccacccgatttgcatgccttaccactttcttttttttttttttttctttgagacagggtctcgctctgctgcccaggctggagtgctgcggcacggccttaccactttctgccatgcgctacttaggaatacgttctccagttaggctctgtagactcagagtaccttgcacactggtgctcattgtgcattttgtgtcatcagtccgctgaatgaacatagtaggaaatcatttttgggaggagtgggatctggggtgataaatcatattttcacttaaattatttaaagtcagtttctctgctggttacaagagtttaagctttggctaacttaataattagctcatgcactaaactggaagctttgattatcctaatgagtgtgaaagaatttcaaagaaaggggagctgtgggtctcgcactgtggtgctgccaagatgtggttaaactcagagcacctgactgtatagttccaagtcgtctttgcagtgcctctagccgagtgatataatctgttagggctctgtcaggatcgtaattctgaagctgagaacatgctaaagaaccaggattgaaatcagctggagtgcctgggtacctattctgaaatggtaaaggggacctaatatagtccagatctgatcttgagcgatacgtagtatgtcttggttctccatataactccagcccaccagaagaatgataaaatgagtcagtcttttctgcaccttgattcagtccaaagccatctctgttaatattgatggaaacagaacctgtgactcgatgccaccgtcgaaccaaaaatttcattctggaaattgcaatggatactctgacggccgaccgaaacctggtgaagccctttgggcgattggtgatcacctctagatccgtgaaagctggctgcccccccatccgggcaagcagggccaaggtggcatcttcacattcctggaacccacccagtaacagcagcaggtatttcttctggtaaatgagagcctttcgaaaactttctgccctcaagtatttaccataaattctctttaaagtgacatgttcagaatcagggctcagagtttgaagtaaagagtcatttcttagttcagctttcagtttgtatacttcagcctctgcccttttcaaagatttctggagagtcaatttttctctgttccatacttctttttcagaggcaatgatggcttcaatgttggcaccaccattcaatgaaaacctggaagaattatctctaccagctcctgtctgtcgataccacctgatctgctcttccagcttcataaccatgttccttaagtcattcttctcttcagtcagttgactgatatgccctgtcagctcagcattttgtctcagtagtctttcagtcaatgagccacaagaagtacttggggacaccaagctgggctcttcaccttgctggccagttaatttctgtagttgtaaaataatttcatcaatattttcctgaacccaaatgaaatcttcatcatctgctgtttcaaactgtagtctctcagaggctttctggggtagaacctgtagttttgaagctacacattgaagcttttgtctgatcatttctaattcatgattacagccggttcctcctccattcatttcaatcaatttagcgtagtttgattcttttgtttctccttctattttctgttgaagaacccaatttctagttctatcactggttaagctccacgtggttggctcattaaggttctgatacagaattcttctactttctcgtttttcttctcgttctagttcttgcttctggaattcctgcatgattccttgtagtcgctgtccttcaaggtctaacttataaacttgttgtcttttctcttccagctggcgctgaagatcttccactttggactggagctcatgcatttttttctgtccctcagtgttggcctcctgttctgtctgcagtgttttcctgtgaacctgcctatctttttccatttgctgtcgtgtttgcaaagaatccagtttatatttttcagtctcatttaacaattctactatgcgactgtgtttttcctctagctgtttctgcagctctttcagtaggtcctctgagggcaagggtggccgagactgtccagtaccatcactgctctgcagctgtgcgtgcaattcccgctccctatctagggtactactcatttcccgaattcgaactttctcagattcaagaagtacctgaagctctaagtttcgaccttgttcttctgacaactgggcatcatatagcattctctgtgattctattttttgctgggattcgttcagtagttgtttctgttgttccaaaagtagatttagctgaagattcctttgtttctgactctcaagtgaaaacttcagatcctcaagttcttctttatcccgttcttcactgcgtcccaacttggctttctctttctccaaagcccactggagctctcttgattttttctgttcacttgctaatgtgtcattaagcaaatgtacttcatctgtcttatctttaacttccaacctgaaagcctccaattcttttaggtgtttatgctgtgccttgagtgttgtttctagttccaatttagtttgtgcaagctcactcttcagttcagcaaccaccattttctcagaactcagctgctcctgcagttccgttgctctgtctttcatactgctgagctccacttgcatctccagcatttgagactgcttctgctgtatattatattccaagagttcttggcttggtttctcactctcttgttctcttttcagagtaattttcctaccattcatttgtgcatgcagtgcctgaatttcagataacaaactccttctatctgctttctggaggcattccatagctgcttgatattcaacaccctgttcttgtattctctgttccaaacagtttagtaaaccaactgcatctgtagtacctagagctgtcagctccgtccgaaatgctgctagtaaaacactacgctcttctaagaaaacttgttgaagggcaagcagtagttcacctcgccagtctgagaagctctcatgagattgagaactatcataaacctcggcttctctttgcagttgcatctttgtaattaaatcctttagagatgagattgtattgatgtaagcttttctctcttctagccaaggttctgaaacctgctgaatagaatggtcctctccatcactatagggagactcagtgagagaaagcacctgcatgccttcattatggacagctctcagtaatccctttattttctttggaaaggaatctgttgcactttcactttcttctcctcggccttctgatgctatgtcaaatccctgactgtgtgtaagataaattccctgaccccagtctgatccagaatcactggagcatatttctctagtctggtaagcatcagaatgtgctagctcaggaattgaggatccctctttacttctcagacactgtatcactgccttcaaggtaccacattcctctttcagtaactgaacggcaacatagtgttccctctttaaggtttcagtttctgaaatatgtctggattccatgtccaaaatttcagcagcatgtagttcttgcatcttctcaattttttcagtaaactgactgattatttcagtaacttcttctgaggaacattcactctgtaaattaatttgtattcctgcatttttaacaagaatttgtggagtctgattgctgctactgatcttcagagtcccatctgtctgggatgcaatgctcttactcagttttataggaagtggctcaaacatgcaggcctttttgctttcttgtacctcagtctcatcttctttttctaaaatggacaatttctcttttgcctctgcgaggtgatccctaacttggcttaagtctttctgaagagatgtcatatttgtttcttttaccaaaagctcttcttgaagtttttcagccttttctttataactggcaagttctgctttggtagccactgattcagctctaagagcctcgagttcattaaaaaatccactttcttcattgctatgaaatagctcagtagttgtcttgagaacttcaacatcttgagggcttcttttcttttctttctctctctgttttttctcattgccctccaatagcttctgtagttctagcagcttcttttctttttctaaaacatttttttctgcaatttctacttgttctttttctaaaatcaaactagtatgcatttcaacaacctggctttctaattctgatattctcaaggttaatgctgatatatctgaccccaactcatcttctcttagttgatttaaattctgaatatttgttctttcaggttctgatgaaattgtttgattatcttgacagaattttgcatattcctgaactgcctcaagttggatttgactgacaagagcagcagccactttttcttcaactattttctgtaggtttacaatcttcttttgaagcatttctgtttcaaactggccttgttcttgcatgtcttttatttgtttataacactgggtaagttctaagtcctttgcactaacagtgctctcaagttgtagcaaccttgtttccaaattaattatggaacctttgccattttcttcaaaagatttgaagtatgtctgattttctagggatttaagagcatcctctgtaaggactacttctagttcaggtttgtctttgctcagatgatctatagccacgttaacactattctctggtatgctttgaatcttttccacactttcacgttctctctttaagctgaataattcctgtgttagctgattcattttaaaattggtttctttaagtacatttttcatgaaggtcatttcttcattagcggtttctacttgctgttccaaggccagcttttcagctataaccacatccaattgatgttttaaactgtctgcttcttctgagagggaatgagcattcattgatgtcttctgtccaatatttgccaattcctgttgaagtttttcaatcacttcattgagctgctctatttcttcttctctatttctcttcacacattcttgatcactcatcaaacattctatttgggtttcaagatcccttatcagttcatttttttcttcaataaccttgttatctgttgtaattttaagttgctgctggagtttcgtaacttgttcatttaattggtcaatttctacctctttttcctgtattatttgagcaaatttcccaaatagcacatgttggtcttgagtagacatggcatcagattcctttatggcaagtcccagtttctccatgtcatccttaaataatttgttttcctgttcaagttcttgtaggcgggtagtagattcctttttctgtatttctaattgcatatgtaattgttgaacttcttcattcttattttccagttcttctctaaactgttctaattgctcttctaagtttgtaatctctttttcctttctgtctatggcatctcgttcagcctgcaattgtacttctagggacaattctggtttagcttctacagctccaaagtgttttcggtcctctaccttttgaaaagtatctgcactcacaagaagcgcctgctccagttctcttactctgaactccagtttctctatttcttcattcctttcttgtatatccctttgaagctgctctttagagagcaaaagctcactgcatttgtctgttttttctttcagatgatttgctaactgttcaacctctctagtttgatgttcactgataggctggaatcgaggaacaaccttaagttgctgttctagtttctgtatttcctgttggaatacatctctctcatgttctctgtcaatggcttgctcatctaaaaattttctcattttttctaactgcttttccaatgcttggttttgctgtcttaaatccattagttcagtatttttttcttgttccagctctataaacctactgacttgttcttccacatctatttctagagctttcacttgtttttgaaggtcatcacgtactttttcagcttgacattgtacttctagtttttccttcattaatttttctgtctcctgtagtaattgttgttcaactgggcctgcctctgctttcatagcttccttttgtctggacagtaattctctttcttcttggatctgctgttgctctgcctccaattcttgcaacctgttacttgcacataacaactcctgctcaagacgatctattatatcagttttttcctgaatttgcctttcaaaaagagttttttcatctgcatagccatcaatgacgccctcagccttactgagctccacagctagctgttctctggccctggactcctcatgaaggcgctctcgaagttcctcttggcacttaagggactctgttgcttcttgtttctgtctaaatgactcacgcatcaactctgtctgtgtcactttcgcatgttcaagtgaataaggaggggtaggcagtgaaattttagaaataagctttaatatatgcccgtttcttttatgaataaaatggaaaatagaagtattaacaattactgagttattttcatccaaatgttcacaaagaggaaaaggatgtggtaaaggcacgcgagattcaacctcataaatgtcttcatcttgctcttctaaccacgagccactgactttgacagttgccaaataggtgctataagaatccatcccagaagatacagctgccgagattcctaatttgctttatcaattttctaatacattaaaaagttctttttagtttatcaagatctaccatagcagtataaaaagtttcttttttagcactatcaaataaatgttataaaattaattcatacaactgcacaataaaaggaaggggaaagtccaggaaaaaaactacaaatctaaaaaaacttaggtctctatcaatcttgatgccccctcaaaaaaacccaaaccaaaacaaaaaccaaaaaaaatcaaaaaacaaaaataaaagcaagcaaacaaaaacaccttttaaactagcataattaagtccttgaagagaagaataaaaatataaacatctaattagacgagcaataaaactgcttttaatatcagcgatgtctgtagtaataagtaagccttcaaagcagaacctggcagggaaggtcaagtttgaaatctccatagcagcagtcttgagaaatgcagttgtaacattatttctcttgctcttgctgcttcactctattcaaaaggaaaagctcttct

SEQ ID NO: 14229 - RNA, 1444 nt, Homo sapiens
  source 1..1444: mol_type = other RNA
gctgggattacaggcatgagccaccgcgcccagccccaggcaacatattttcttaaggcagctttaacaggccatgcatttccacatttccacacctttgcatatgctgttcactctgctccaaattcccttccctgtttctctcccgcacttcaccttccttttaactttttcttcaaactcagctcacgtgtcttgcttagggagggcttccccgacctcctcctatcccagactgggtaaggtactcctggtctagcagcatccttctgtttaccttattcttgtagctctagcaccactaaaacgtttttcctgtaaataacataggtgcatttttaaatgaaaccgtgaacaagaaatcaccctaattccgtcggcaatttattttagtatttcagtagagttgcttttttaaactaaggtttggaagtctagcttccagctgcaggtttgtgagcatcctgaaattcagttcttccaccgatgcgtcaaaagacgcgacagaacagtggacctcgaagccaggacctaggtaagggcagggcctagctctagctctgccacccataaattcacatccaccctgtgcctgggactcagcttagccacacacaccggccccacccctccggggtctctttcacctgtcacccgccattaaccccgtcagcttctctccaatgacaccccagggttgtcctacagggccaccgaagcctgaagctcctgtgagtggggccgataagaggccattttgaaaagtcctcagcatgggcttcgcctttagatccacgtcgtttctcctttctaacccgagatgtgtcccttgggtgcgaagcgacaccagcgattctctcggaggccccggtggctcacccccacgactccccggggaggcggtccccatccctagggaaacccggcccgcccagcctttgttgcagaaaccgcacacggagccatatttgctttcagccaaaggcagacgtggtcggaggagtcggaagggcaggggcggacccgaaacccgccgtgcgccccacttctccatcgcgctccttcctggactctgaggaagagaaaatgcgctcgaccacctaaggaccgcgtctccaccttccaccttcccaatcatctgcagcttcccaatctgcagcaaggtgtcacaagggcttctccgcagctatgatttctaacaccatgccccgggccaggagcctcagggtgcccgttcgggaaaatgggagccgaatcaggatcaccccatgcgcccccgcacccttcccccgccggttccaacgcccgggcgcccctagaccggggggggggttctgaggtggacttcctgcgcctcctcgcagcttccctccaactccactaaacgggcacagagacgccaccgctgtcccagaggcagtcggctaccggtccccgctcccga

SEQ ID NO: 14230 - RNA, 9315 nt, Homo sapiens
  source 1..9315: mol_type = other RNA
gctgggattacaggcatgagccaccgcgcccagccgatcttttgttttttaattattattattttttttgatacagggtctggctctgtcacctaggctggcacaatcacagctcactgcagccttgttccccagcacctcagcctcctgagtaactgggaccacaggcatgcaccaccatgcctggctagttttttattttttgtagagaggggatctcgctttgttgcccaggctggtcctgaactcctgggctccagtgatcttcccgcctgggcctccaaaagtgctgggatgacaagtgcgagccaccacacctggccccaatttagctctgtttcccttcctcttcctctcatgatgcttctggtagattccatccatttctgagggatttcccctgaggttaaaactgccttgttttcctgtggcttagttgtcattatcatatgatggtagtattttcaaccatctcccttatcctctgtcctctgtccagatggttctgtctgggccgacggcacagctgtcatcccgcaacttctctttatcctgggctacaatccagtcctgcctcacacgtccttctctttattattttactccttatttgtgcagttggttgttatgtggacttgtctagttttggtaaacacctacggtcctataaccaccaccactgtctggcaccgtggccccacagctggacggctggagctggcagcttttaaacccaactcaggtggctgtccaagccaccctatttaaaattgcatctcaaaaaaaaacaaaaacaaaaaaagaagaaaggccaggaacagtggctcatgcctgtaatcccagcactttgggaggctgaggcgggcggatcacctgaggtcgggagctcgagaccagcctgaccaacatggagaaaccctgtgtctactaaaaatacaaaattagctgggcgtggtggcacatgcctgtaatctcagctactcaggaggctgaggcaggagaatcacttgaacccgggaggcggaggttgcggtgagccaagatcataccattgcactccagcctgggcaacaagagtgaaactctgtctcaaaaaaaaaaaaaaaaaaaattgcatctcacttggctgggcacagtggctcacaactgtaatcccagaattttgggaggccaaaacaggaggatcacttgagcccaggaggttcaaaaccagcaagactccatctctactaaagaaaaaaaaaaaaaacaaaaaacagctgggtatggtggcaagcacttgtaatcctagctactcagaaggctgaggcaggaagatcacttgagcccaggacatcaaggctgcagtgagttgattttgccactgcactccagcgtgggcaacagggcaagatcccgtctccaaaaaaaaaaaaaaaaaaaaaaaaaaaaaaggtcaggcatggtggctcacgcctgtaatcccagcactttgggaggctgaggcaggtggatcacgaggtcaggagatcgagaccatcctggctaacacagtaaaaccccgtctctactaaaaatacaaaaaattagccgggcgtggtggtgggcacctgtagttccagctattcgggaggctgaggcaggagaatggcgtgaacctgggaggcggagcttgcagtgagccgagatcatgccactgcactccagcctgggcgacagagcgacactccgtcaaagaaaaaaaaaaaaacataaaaagtaaaaataagattccatctcacctggccgggcacagtggctcatgcctgtaatcccaatactttgggaggctgaggggtgaggatcacttgagaccaggaattcaagaccagcctgaacaacatagcggcaacctatctcaaaaaaaaaaaaaaaaaaagcctggcatagtagagtgcactaatacacccagctattcaggaggctgaggtgggaggatcacttgagcccaggagtttgagactgcactgagctgtgatcttgccactgcactccagcctgggcaacacagctacactctgtctcaaaataaataaataaataaattgcatgtcaccttctccccacctgcattacttaacaggcctgggagtaagactttggtaggtgcaccatgatgggtgccacaacctcgacagtatgcaattgtcaggttttgaaggagctggctgcagctgaaaccgccggagggttctaaacagtgaggcaacatgatccaccttatatcataacaggatctctctgcctcccacgctgagaacaggctgaagagagccagggcagaagcagggagactggcatccaggcagagatagacgatggcacaggagagctgggtgggggtggtggaagggaggagaatctatctaccttgaatctgtcttgaaggtagagccaccggggtttgctgatgggtcgggtatggccctgaacctccccaaaccctctgggaccctgcaaggagtggtcctttctcccacaatggggctccagctcatgcagcatccacaggtctactgacctgccccaaggacagagccccacatggatggcatttccccaacatttaatcaggaaaaaacattccatgaacaaagaaaaactcatgcaactaaagaggagagaacggggggtctgggactgtcagacagggccagattcctcagaggaggcagaagacacagagtagtaaggcacggccgccttggccccacagggcgggcactggacggagcgggcgctgaatggggcggctgaaggagtcggagcaggtgcagacaacactgaggacgtttggcagtaggctcaggaggaggagcgttctagggcccccaggcccaagtcaggccctggcacaagcctgagtccagccctccaggtgctcagagagaatagggccccgagatgcttgagggggaccctgtggtccagcgtggcacagccacaattctgaggaagctttggaggcctcaccccaagtgctgctggtaccgtgaccccgccttggaatgggtggggtcagccatggcaagggtgaggtgccagaggccagaccgaggctgataatgctacacaaaggagcccagacgggtggcagggcccaggacagctcaagaagaggcaggtgagtgagggtggcgacatccggtggggggacacatatttacagatggagacagaggcgaagttcgattcaataaataggcagagggatataaatagcagggagggtgggactgtcccaacacctgggcacagggcaggagggtgggggtattgctgctgctggggtgggggctcgccctgtcacccctccccctgcagggcccaaagcaaggcactaatgaagggggcctgggtgtgccgggggcatcgtggccagggtgacctgccccacgatacccaatccagggctcagcccggggacccaggcttgagccagccactcccctggatgggaggacggcacaggactgagaagccccctcctcaccgattccaccaccttagctgtcgctggacacgaggctgatgatctgttccagtttctgccgcaacttatgcttccgacaagaggcatctcggtccagagccgtgagaatctcctggcggtacttggtgacatagaaatacagctcgttgagcgcactcaggacgctgaagtcgctggcgtggaggcgggactgctccaccaggtaggcatccatgtcctggtcgctgatggatgccatctttgcaatgtctcgataatacctctccacccagctcttgtagttggggatgtccttggcgtagagcagtttgttggagggcgagtccttccccaggcggtgctcggatgtagagcaggagtccatgaaggtctgggctaccaccgacaggcaggcatccgtgatgctgttcttgtggatgtcgaacacgaactgcgggttcttgatcacattcacccagaagcgcagcggcaggcagttgctcttccaggtgtggcgcacatcggggtcgctgatctggcgctggtccgcctgctcatccaggaagtcgaacatgtacttgatggccaggggcagggccgagccccggtgggctgtgctgaacactgtctcaaagaggtcatccacgaacttctgcagtgtgcccttggtggccagcagccgtgtcaggtagatctcggagaccatcttgctgccacggtccccctcgcgatggtcggcatggtcgtggtttttcaccaggtgccacaatttggtgcctgtctcctggtcaggcgtaatcatgggtgcccgtgagcggaggctatcagggctgctggccgtgcggagcaagctctcgtagcggctgagggagcgggtgaaggtgaaggagttggccatgttataggcagacacttgtttgggcaccaatgccaccaaggaaccgtctgtcacctggtagtgggccagtgagttgagcctcttccagtcacactcgatcttggtggtgacatcctcatcctggaggatgatgcgagtcatgcggccctggcgccactccaggtccatgtcctcagctttgggacgctgggagtacggaatgcccttgtacacagtgtccagcagcttatctttggcctgggtgatgctgtcacagttgagaaccttcactgggacctgggcgctgccctcgttctccggacacacgcagtgaagggtcagtgtcttgtagtcgatctgctgacggatgagcttgtcctcgctcagggagtatcgtgcctcgcccgtgatggcatcaatggggcccttctccatctgctgcttgatggcacagtaaagcaggaagagaggctccccagcacactccttcagaaacttatgcagcaggaacgtgaaccagttggtaagcatcttctcagccactgactctgtcctgcgtagcagcagcttggggtggttcttgctctcgaggttcttctcgatgaggtcggccagcagttgcttgagcagccccgtggcatagtcgagccggctctgcagggccaccatggtgagcgaggccacggtgccgcggtcgcgcatggagaagctgctctgggcctccagcgtgtggatgaaggtaagcacgaacgcgcggctgtgcagcagctgcccgaagaggcgcagggccttctccacgttgggtggcgtatccagctccttgagcaccgggtgggcctcgatgcccgggaagagcacgcgcacggcgtaagtccggtagtccaggaaggggatctgcacctcgtccatgtggttagtcagctcattgatgtccgtctgcagctctgcaaaagcttccttgcactccagggccacacgggactccaggttgtccatctgcagctgcagacgcttgagggtacggtccgcgtcctgagtcttgcgcttgtaggccaccagcacggctgtgatggccagcagcaggagcccaccccccgccgccagccccatcatggccggtagggtcagcgcccgctctgccgagatgtgcagggtgcccagccagaactccaggccacccaccagcaccatgacaggctgccggccagtctggctgggtgagtcgcacaggagttgtgtgtccgagacagtgagcgaacacggctggcctcctatcagcacagtgtagttgaggcgggagctgccggctgcagcgggaatcaggttcttgcccttcagcaccacgtgggagcccggtttgacgtccagcacgccagagggccccagcggctcaaagctgggatcagggtagtaggtaaaggaggagcggttgagggagcgggccgtttgcacgtggtccagcaggaagccaaactcatcagggtgctcgccttgcgcccgaggctggggccgcccaagaaagatgccgggggccttacacagcatggcagtgtcgttgatcacttggcatgtattggtggtctcaatgccgcggtacttggcacggacccggggctcctggaccgtcagcaggtgggtcccactcacagtgatggcagtgcttccattgatgatgctccaggtgggctcaaggcgggtgacggtggggtcctgagtgtaggtgtagatgagcccggggctggagatgttagcccggtcaatggcaagtgtgatgggggcctggctggggcccagggtggagagaggtgagatgcacacgatcgccttggcatctctccttacaaactggcactcgctgtccctcacagtcactgtgaccctgctgccagcatccagagagctgcctgagatggtaagccgtgtgcccccggacgccgggccacggctgggactcacttggtcaaacgttggggtcacaaagctgtagacctgctccgactgcgtgcggaagtcggctgaacagtcacccacacacagctccacgggccccggcggcgggctgggcaccagcgactcctccatctcacacacgatcctctcagcactgatgtactcggccggaatggagttgcaacgcacgccagccacccgcaggcccacctctcgggacaagaggcccaggttctcacccacgatggtgacccgggtgcctccttccttgggccccacgagagggtggatctgcgtgatgcgggggtggctgcaccgggtgcccttctggctcaggtgcatccagttggtcttcggggccgggcagtgggtccgcagctggcacctgtgctctgagatgcaccagccacagttgaagcggggatcagccttgaggcagaggccacagctgggccgctgcgcccagcacttgtacaggagggctcggaagctgggaggcttgtctatggggaagtctccatcccagaccacggaaaagtccagctcggtgtcaccatgctcatcaccttcataggagtacgaggcgttctggcactgcacactgctgctgttgaagcgcacggcaggcacccgctgctgccgcccctgcacccgcaccacgcactcatagttcttctggcccgactgcggctgaggtaggttcttagcccgcaaggtaagaggctgcatgaccccaacggggatcaggaggtccccactgggcaggatctcagggcagccctcagggctgtggaccctgccctcctggaaggagcactcgtgggggcggctggtacacgtgtggcggtacttacaccagtggcaggggtaagggctgccaacacaggacatgcacgactggaggacgctgcagttgtagaagacaaagtcagcaccggcaaacctcacgcctgtctccttggagagaagctgcagccgcacagtgcgggtggccccatgccccctggtaagagctcggagctcctggagggagggtgaggggcagagcagttcaccggagggcagcaggaccgcctcgttctccgccgccgcctcgaaggcgcagctcacgcccgcactgaggtctggcacgttgtgcagggtgacggtcagctgcaccccaggtgacgtcactgacacattgttgggccggacccgcacctggacacacttgctcagctcctcagcaaagccgtgtggggcagaggcgcccagacaggccccttcgcggcagcacctgtgtcgcagcacacaccaaccacagtgcgggtccccggagcccaggcaggctgcgcagctctggtactgctcacaggtctccaccgggagctggctcacctgcttctcactcaggagatagatgtgccggtggtccgggctgaagagcaggtctcggaggatggggctgccatccaccacggggactgtctcatacaggtgggcatcctggaagccatcgacccgcaccttcttcaagctgccgctgcgcgtgccaatgaagaccacagagtgctggcggtaggtgtaggcggccacgctggccatgccgtcggtgctgtcggccagcaggggcagcccctcgatcacatgcaggcctcccagaggctggttcaacaccagcccacagaagttgccgttgatctgcatgggggtgttgatgcagggcagctccttgttcagcagccagggcagagccagagtgccctccccacgatagcaggactggatgcggcgccggatgtgggcattgatgttgctgagggtgaagaggcagaggatggtctgccggggtgggctggcccggttcttctggccctgagagaagatggtgaagaggacgtcctcatcagccggcacgcccagggcctgggccagcagcaggccaggcttggccaggtgggcgctctgcaccaagcggtactccacgccgcgccaggagcagccgatggggaattccacgtatgagtagaactctgagtctcccgcgcacatgcgcacgatcttggacgtgaaaaatttctcgcccgctgtgtccaacagcgtctgctgggtgtccagctgcagcgtcaggaagtacacgaaggaggcgctgacgaagccgtagatgtagtagatgtcaaaggcagggtacaaggacagcgtgtctgaggggatcttgatctgggaggacacaaactcatcctggtacacgagactgaacatgtccgcgctgtcttcatcactgatgagcttgcgggagctcaaggtggggaagtactccgacttgccgtcgacagcagtgcccacaaacagcttgctgggcccctggccctgctccacaatgacaccagccatggagtcgggctcctgggcccccgacaggtagtgctccttgcggtggtgcggctcacccagcttgaagaggtcgtccagacgcaggaactggcagatgccctgccagatgctgccgcaggccaccaggcggcgggccgcatagtctatgagcagcagcttgttgatgttgtccacgggggccaggcggtgggcacacacgcgcatgctggggggcgggtagcagcgagcgttgtcctcgacgggccccgtgacatgggcccgcagctcagtcaggttgggggccagcttaaagactcggttcactgcgcccacgaacacctccccagtcacccggtgcacagccaggtgggtaagcgtggtgtctgtcaccacgaaggcacggaagggcctgttgcccagggccccccccacggcaaggaagagcagcaggaggaggcagacagagggcatggccggcagccgcgcctggggacaggcctgtccctccgctggctccgggtggccgccctctggccacgtggacgcgcccccgagccccaccgcggccccgctcgcacgtccccacggcctcgccccgcgccccgggccccaagcgcgcagccgccgccgccgccgcccacacact

SEQ ID NO: 14231 - RNA, 1093 nt, Homo sapiens
  source 1..1093: mol_type = other RNA
gctgggattacaggcatgagccaccgcgcccagccgcccagcctcttatttcttaaatgggaataacaatgcccatctggaaggatgtttaggaggcttaaatgcagggtctggcacaggccaggagccagataaacctgagttcccttccacagccttctctctcttccctccatcatgccagcttcccccaagcatggcacaccagaattcaacttctcccctgccaggagagcaatttccagaagttccaggtaacatatcagctcccaagccagggccaggccacggtctcttctgagaggaggaaatcttcagggccaggagcggtggcttacacctttaatcccagcaatttgagaggctgaggcaggaagattgcttgggtgtggtggctctcacctgtggtcctggctactcctctggtggctgaggtgcgaggaacacctgagtccagggaagtcgaggctgtatgtgagccatgatcgcaccactgcagtccaaccttcatctccgcacaccagcttcttggccacacaggggatctcgacatagccaaaggccttgagctggtctacctgctgcgctgtgatcgggtgctcccacatggcggtgttcatggccgggcagaagagcaggggcttgctgcggtcccaggcccgcatgacgcaggtaagcaagttgtcacagatgccactggccaccttccccagagtgttggcatcaagaggagccaccagcaggaggtctgcccacctccgcaggtcaatgtgcagaactgggtcagagcggctcttccatatcccaggaatgtccaaaagctttgacaccagaagaggcaacttcagggctgcgacactccccgtgacacccacaagaacatggaattttctctccatcaagggtgcagcagctggacaggaggcctttggttccatgtggggtctggtggcttcaagttctgggagcctgccaggcctgggctctataaagctgtcgggatttaggatccgcgccaggcgcgtctcggggccgctcccaaatatcgcggtatctctgccgctctcccgcggaatctgactggcacgcctca

SEQ ID NO: 14232 - RNA, 1133 nt, Homo sapiens
  source 1..1133: mol_type = other RNA
gctgggattacaggcatgagccaccgcgcccagccgcccagcctcttatttcttaaatgggaataacaatgcccatctggaaggatgtttaggaggcttaaatgcagggtctggcacaggccaggagccagataaacctgagttcccttccacagccttctctctcttccctccatcatgccagcttcccccaagcatggcacaccagaattcaacttctcccctgccaggagagcaatttccagaagttccaggtaacatatcagctcccaagccagggccaggccacggtctcttctgagaggaggaaatcttcagggccaggagcggtggcttacacctttaatcccagcaatttgagaggctgaggcaggaagattgcttgggtgtggtggctctcacctgtggtcctggctactcctctggtggctgaggtgcgaggaacacctgagtccagggaagtcgaggctgtatgtgagccatgatcgcaccactgcagtccaaccttcatctccgcacaccagcttcttggccacacaggggatctcgacatagccaaaggccttgagctggtctacctgctgcgctgtgatcgggtgctcccacatggcggtgttcatggccgggcagaagagcaggggcttgctgcggtcccaggcccgcatgacgcaggtaagcaagttgtcacagatgccactggccaccttccccagagtgttggcatcaagaggagccaccagcaggaggtctgcccacctccgcaggtcaatgtgcagaactgggtcagagcggctcttccatatctcccattcatcagcgtcgctgtagagggtgacaggaatgtcctgggggctgtagaaatgtttggctctctcagttgtgaccactgctacttccagcccaggaatgtccaaaagctttgacaccagaagaggcaacttcagggctgcgacactccccgtgacacccacaagaacatggaattttctctccatcaagggtgcagcagctggacaggaggcctttggttccatgtggggtctggtggcttcaagttctgggagcctgccaggcctgggctctataaagctgtcgggatttaggatccgcgccaggcgcgtctcggggccgct

SEQ ID NO: 14233 - RNA, 1540 nt, Homo sapiens
  source 1..1540: mol_type = other RNA
gctgggattacaggcatgagccaccgcgcccagccgcccagcctcttatttcttaaatgggaataacaatgcccatctggaaggatgtttaggaggcttaaatgcagggtctggcacaggccaggagccagataaacctgagttcccttccacagccttctctctcttccctccatcatgccagcttcccccaagcatggcacaccagaattcaacttctcccctgccaggagagcaatttccagaagttccaggtaacatatcagctcccaagccagggccaggccacggtctcttctgagaggaggaaatcttcagggccaggagcggtggcttacacctttaatcccagcaatttgagaggctgaggcaggaagattgcttgggtgtggtggctctcacctgtggtcctggctactcctctggtggctgaggtgcgaggaacacctgagtccagggaagtcgaggctgtatgtgagccatgatcgcaccactgcagtccaaccttcatctccgcacaccagcttcttggccacacaggggatctcgacatagccaaaggccttgagctggtctacctgctgcgctgtgatcgggtgctcccacatggcggtgttcatggccgggcagaagagcaggggcttgctgcggtcccaggcccgcatgacgcaggtaagcaagttgtcacagatgccactggccaccttccccagagtgttggcatcaagaggagccaccagcaggaggtctgcccacctccgcaggtcaatgtgcagaactgggtcagagcggctcttccatatctgccctgcccaggccaacctccgttccctcctgcagctaagctggcgagcgctagccatggagccagcagccgagagaaccaggcctgaggaaacaagtgccccttgtctctctgagctattcccttcatggtttggctttcaagagaactgacatctggcagggagctcccggcctgtctgcttgaggcggatgcttgggttgtccaagccagtggaaagctccggggcagtgagaaatggagggggtgggggcggggaagacaggccagccggaaatgttctaggctaagaatgtttgaaaatgcctggcagggaacccctgtgaggcccacactcagcgtctggtgaatcagccagtgcccacccatccgcaggggagatgcagcagagcccggcggccgtgggaagtgaggcgttctcttcagccctgacgccaggaaccacgtggacaagggtggtgggaacagagctcctctgtggtttcatcagcccagataagtacaaggacactcaacctcaggcaccaggccaaagcccagctctgcctgggccgggaggagactagggcctcctgcaggccagaagctagacagatgttttcttcattgcctctgcccagagggccctgaccacagacttgagcccagcctgtctgttccagctgccagaccataggccgtagggaggactgttctgtcctgctggtggaaactcaatggaactcagcccagggg

SEQ ID NO: 14234 - RNA, 964 nt, Homo sapiens
  source 1..964: mol_type = other RNA
gctgggattacaggcatgagccaccgcgcccagccgcccagcctcttatttcttaaatgggaataacaatgcccatctggaaggatgtttaggaggcttaaatgcagggtctggcacaggccaggagccagataaacctgagttcccttccacagccttctctctcttccctccatcatgccagcttcccccaagcatggcacaccagaattcaacttctcccctgccaggagagcaatttccagaagttccaggtaacatatcagctcccaagccagggccaggccacggtctcttctgagaggaggaaatcttcagggccaggagcggtggcttacacctttaatcccagcaatttgagaggctgaggcaggaagattgcttgggtgtggtggctctcacctgtggtcctggctactcctctggtggctgaggtgcgaggaacacctgagtccagggaagtcgaggctgtatgtgagccatgatcgcaccactgcagtccaaccttcatctccgcacaccagcttcttggccacacaggggatctcgacatagccaaaggccttgagctggtctacctgctgcgctgtgatcgggtgctcccacatggcggtgttcatggccgggcagaagagcaggggcttgctgcggtcccaggcccgcatgacgcaggtcccaggaatgtccaaaagctttgacaccagaagaggcaacttcagggctgcgacactccccgtgacacccacaagaacatggaattttctctccatcaagggtgcagcagctggacaggaggcctttggttccatgtggggtctggtggcttcaagttctgggagcctgccaggcctgggctctataaagctgtcgggatttaggatccgcgccaggcgcgtctcggggccgctcccaaatatcgcggtatctctgccgctctcccgcggaatctgactggcacgcctca

SEQ ID NO: 14235 - RNA, 2425 nt, Homo sapiens
  source 1..2425: mol_type = other RNA
gctgggattacaggcatgagccaccgcgcccagccgcccagcctcttatttcttaaatgggaataacaatgcccatctggaaggatgtttaggaggcttaaatgcagggtctggcacaggccaggagccagataaacctgagttcccttccacagccttctctctcttccctccatcatgccagcttcccccaagcatggcacaccagaattcaacttctcccctgccaggagagcaatttccagaagttccaggtaacatatcagctcccaagccagggccaggccacggtctcttctgagaggaggaaatcttcagggccaggagcggtggcttacacctttaatcccagcaatttgagaggctgaggcaggaagattgcttgggtgtggtggctctcacctgtggtcctggctactcctctggtggctgaggtgcgaggaacacctgagtccagggaagtcgaggctgtatgtgagccatgatcgcaccactgcagtccaaccttcatctccgcacaccagcttcttggccacacaggggatctcgacatagccaaaggccttgagctggtctacctgctgcgctgtgatcgggtgctcccacatggcggtgttcatggccgggcagaagagcaggggcttgctgcggtcccaggcccgcatgacgcaggtctgagcagttgtgaaaggagccatccagctcacagagtcctttgtgccacggactttgaaattacgtagccctgagttcaaatcctgactgtgctctagctgtgagagcactagctgtgtgtgtattactagctgtgagaacctggacatgggactgaaggccagggcctggcttcctctctagaaaggtccctccctgggcagctgtgaggactgaggtgagaatggctacaaagctctgagcgcagggccaggcacaaaacacaggctccagggcagtgactcctgggcttcccacaggcacaggctccctgggctgggggccgcctgggggagagagaagctcccagtgctctgactactccagacacctcttccagggctgtgagctcctcagggtaacaggctggaaacccctcccctgaagggaagctcatctgggaaaagagcgaaggagtccagagaacaatgccccgacaggacaggaccagcacctcccccaagtcccagggacagggaggaagcaggacagcaaacagccctgggacctggctgcttgcatcagccaccagcattagtttcccaccaagccctctcaatacggcagccgggctatgagtggacagtttcagtcacacttcctcttggctccatgccacctgctgcttctgcagaaatcaagagcatacctagaaaagtcgctccgctgtgtgcagggcaggagcaagggctgggctgggctttctaagtgccctcaaagcaaagcacaccaaccagggtgaaaaccagcactccaactcctctcagacaagcctcagctactctgaacccacgaaagcaggcaggaggagaagagagcctcggttcccacggtgacatctctttggccagtgctgtgttcaacatttcaggctctgcccctgggaattcacatgggcaggggagaaggcctggatcccagtcaggagaccagctcctagccagactggtgacccagagagattgtctgctctttctaggtccgactgcctgtttagcacaaatgggccagggccttagtgggctagaggacagagggacacgggcctggaggccaggagcacggtcacacctagcatgctgccctcacagcaccccatgccctgggcgctggaaagggaggtctgcggatggaggagcaggctcaacttcctttcagggatgtagggagaaaacagctacagagagaggacacagccacaggccaccaatgcccacacttcaaactttgtaaaatttgagattccttgaaacatttgtgacttcgagggaaaacctttgaggcaaatgatctgggggctggtcttgggaacatgtttcacttcccagccaactctggaggagggaagcccagggatttcatgaagtgatggcagcttagaaggaaaaggggaagcagagcttgcaggaagaaggaaagcgcccttgcagagctggcccaggccggggcttagctcccagaggccagtactttgtcacaccagctgctgctgacccgccagcagggagcctggagatttggtgagatggtgctggccacacacaactctgacccaatttgatgagagcagccaagaaactcaactgttctagctgcagctgccatgtcagttgtggcaccagtgctgctgggaagcctttttgtttttttgagacagagtctcacctctgtagcccaggctggagtacagtggcacaatcacagctcactg

SEQ ID NO: 14236 - RNA, 2265 nt, Homo sapiens
  source 1..2265: mol_type = other RNA
gctgggattacaggcatgagccaccgcgcccagcctaataattttatttcttgttcacatttgtctgatgtaggccaggtgactctcttgggtatttctcctctaggcagtggctcagggctccccaggtgggtggaaaatggggaacatggaagatgaggagtgaggaggggcctatatctgtatctttatctcatacacccccccacacacacacagtgacatatataaaatatgtggtgacacatataattttgcttttagttcaatgaaaagcacatatagatatatatagctacacatccatatcatacatatattgatatgtatagataatacatctctatatgcttttcattgactaaaatcaaaattgtttttaatttaaaaaaatttttagagacagtgtctcactatgctgcccaggctggactggaactcttgggttcagacagtcctcctgagtagctggaactagaggctcacatcaccgttagaaaacaggtttttaaattctgaaacttagtctgtaaattcatctgttgattcctgggggctcttgaacctcaggaaatgctgctgtgattattaatattagctgagactctggcatgtaggaagtgttacatagttgctattgttatttctgtcagggattctcagtgggaataatttacactaaggtgagaatggggtttaaccttcctttgagttattttttattatataattaatatgtgtccattatagcaaaattgggaaatagatctgtttctgcatataaaagaaatttttaaatttgtcttcattccatcatgcaaaggttgtgaattatattttataattatttacattttttaaaggggaactaattaatgaatttctcattggaaaattattctgtggagggaacgtgaaattggatgtcttctgatgttcttactaaatcaggactagatctatctagctttccctctagaacccctgggccccaggaatcccctggatagagttgttgttcagggaaggagaatggattattctaacaacttgcaaattaggagcctggtaatggaaactgcctcttttaacaaatcttcaagtggattcctaagctatccattgttcctgattgattttggacagagcaaatatatctataaatgggaatccctaacttgctgactactttgagcttaagcagtaaagatgtttggatatcagtagtgtcagagaggagaagtagggagtgggaggaatgggaaggtttttggctgacccccaaaaccagataaagagctggagctcagatagtgcccagcatctcaagaagtgtttcttgccagcagtgaccaagccaaagcctactgttcctttagacaaagtaggacaagggagaatgagatcttgagtgggctaagtgcctctcaaggatagggacctgccttgttcgtctccttctcccattcccaacacagacctaatttagtcagaatttgtgagactgaattgagttcaaaagtggcaatgacaaaaacaactgtggtagtattattaccttatatgtgttgacattaaagtttcatgccaggattctactctggagtgggggaagaagggcattaaaggaaaaaaaaaaaagtcaaggccaataaaatggtcagaatctccttaggttagaagtcagagcagttaaactgtctcctatatatatatgtattttcctttaaatatttgatatattagaggaacatgaggaaggaacagttctaaccaagagctctttgggtaacagctgtcaggtaacagtggaaggtcttagcccagaagctgggctgccttgggcaggctcccagagactaccttggcttctcttggctctgcagaaagggaacgatgagctgcttttttaaagaggcgtgccctaggttcattcatgctctttactgggcttttcagaagagtggggagttttagtttaccttcttgatgataaatccacagtataccccaagtgaccagacctttattaaagggtgtcattagcttgaagcctttccttctgttatatgctattgccttgtggtctcagaatgatcactatcgttaacattcacgggtggttcacttatcattcctgactgcacagacatggcagccgctcggaagcgtccgcaggtgtagcatggtgatacatattacattgtgccacaatggatttatgtatttttaaaacttgcttaaacacggccgggcgcggtggct

SEQ ID NO: 14237 - RNA, 2342 nt, Homo sapiens
  source 1..2342: mol_type = other RNA
gctgggattacaggcatgagccaccgcgcccagcctcaaaactttcttctcagttcacattccttcctttctgccaatgccagtagggtgaatcagataacctagagtggtgagctagctaatatggcagtgctgtccccagaaactactggaataagggggaacatcaggcacctacaacctggagagaaagacttgtcaggcaggtctgcttcctgctgccttgggcacttccttcgggactggtttgttgagagggttgagaatggattggaggggggggtggggatagtgggggaactagaggcaggaaagctcatcaggaggccttgctgcacttccacatagatgggggcctgacctgaagtagtgaccgtgcatggagagcgaggttgttgaagtgaaaacgtgaaggctagaacaggcctgacttgatgactaggcctatgggagtgtgagacgagggtgtgcccagatttcctgcttggccaggtaggtgagtggcagtgccacttattgagaaagggatcatcaggcaggacaaactgtgagtttgagggggaaggaaaggatgacaagttgtgttgggtagattcaatttgagttgcctataggatgtgtaagtggggctgtccaggaggcacttggatgggagtgtgtgtgtttcgagcacagaagcaaagtctagtctggaaacaagagtattaattttctctctctcactgtttctctctccttcacacacacacacacgtgtgcgcgcgcacacacacacacacgtgcaaacaccagaactttcaaagctaggtgcactcacagggtcattaagcccaggacatgttgacaagggtgtggaggtgtcatcctcggggacatgcagggagggttcctggacagtgatttttacatcgcctccttaattgtccataaccataaccatgatccatagccataaggacaataggaattgtggtcccccagagatttttttcctactgaaactccatagtcacacctctttgcagactttatggcaggccttcccttttttccaaacccctgtgaatagtgtcagacagcatctgcgggaggatgtgtgtgaatgctgggatgcagggggcatggcagggagtggagcacttgtaattctgttgatgttggagccctcccctttcagagtgcattgagtccttagtgtgtgccccctcgccccgatcaattcccaatccctgtgttgcagagagggcagcaccaccttctcagccgcacaggatattctcaggctgatgccaagagcaaatcactcccagccagcacacttctgccagccttggtaggcacagcgtgtagcagtgcgcatgtgggtggggacagaggtgacttttctcatagactgggagaaaaaaaaaggcatctgaacttcctggttacagaacatccggctagtagaaacctttgtgtgtttgtacgtgtcgggcagggggggattagtgaggttcccctcccctctagtgttagcaataatgaaggacactctttgtacaagacgtcaagatgagagcttccacacaggactccacactgtgcttctgtttcaccaggaagaaatcttgaatgtcagccaggcttgtactcatcaattcattcagccagtctctgagggctggtccttctactgagtgctggctagggtggggctgaggactgtgcccctggagagctgccagcctaggtgcaaacacagaaccttcattcatgcagtgacatcacagcagcccatcacaacactgccccaactgcatcagagcagttgcacctgataggtttcccaggggttacctgaggagcaaagccaagtgcgtgtggcccaaagtagacagcatatagggcctgcacgctgaggactgccccaaatgctggcccagctttttccaccagggagggtcagattccaaagccgacagccactcagcacgaggcccagacccaaattccactgccagccacttctactgctgtgctcttcagatgatttatgtctacagtatctgtagagttgaaatactgtataatagtgtgcaattgtgtctcttcccaacatcacattgaagttaactgcttgaaatcagccacagtgggaacacttacaactcagaaatcagcaaatgctataaatcaggcttgatctattcttttgttgtctatctcttgtgggcagagtgtaaatgcactgcagctggacagcctcagagggtgcgggcttcagccagctcctcagtttgatttgtctctgacaatgctggagtgtgctggtctcttgacctcgctgcgccttggtttcc

SEQ ID NO: 14238 - RNA, 2231 nt, Homo sapiens
  source 1..2231: mol_type = other RNA
gctgggattacaggcatgagccaccgcgcccagcctcaaaactttcttctcagttcacattccttcctttctgccaatgccagtagggtgaatcagataacctagagtggtgagctagctaatatggcagtgctgtccccagaaactactggaataagggggaacatcaggcacctacaacctggagagaaagacttgtcaggcaggtctgcttcctgctgccttgggcacttccttcgggactggtttgttgagagggttgagaatggattggaggggggggtggggatagtgggggaactagaggcaggaaagctcatcaggaggccttgctgcacttccacatagatgggggcctgacctgaagtagtgaccgtgcatggagagcgaggttgttgaagtgaaaacgtgaaggctagaacaggcctgacttgatgactaggcctatgggagtgtgagacgagggtgtgcccagatttcctgcttggccaggtaggtgagtggcagtgccacttattgagaaagggatcatcaggcaggacaaactgtgagtttgagggggaaggaaaggatgacaagttgtgttgggtagattcaatttgagttgcctataggatgtgtaagtggggctgtccaggaggcacttggatgggagtgtgtgtgtttcgagcacagaagcaaagtctagtctggaaacaagagtattaattttctctctctcactgtttctctctccttcacacacacacacacgtgtgcgcgcgcacacacacacacacgtgcaaacaccagaactttcaaagctaggtgcactcacagggtcattaagcccaggacatgttgacaagggtgtggaggtgtcatcctcggggacatgcagggagggttcctggacagtgatttttacatcgcctccttaattgtccataaccataaccatgatccatagccataaggacaataggaattgtggtcccccagagatttttttcctactgaaactccatagtcacacctctttgcagactttatggcaggccttcccttttttccaaacccctgtgaatagtgtcagacagcatctgcgggaggatgtgtgtgaatgctgggatgcagggggcatggcagggagtggagcacttgtaattctgttgatgttggagccctcccctttcagagtgcattgagtccttagtgtgtgccccctcgccccgatcaattcccaatccctgtgttgcagagagggcagcaccaccttctcagccgcacaggatattctcaggctgatgccaagagcaaatcactcccagccagcacacttctgccagccttggtaggcacagcgtgtagcagtgcgcatgtgggtggggacagaggtgacttttctcatagactgggagaaaaaaaaaggcatctgaacttcctggttacagaacatccggctagtagaaacctttgtgtgtttgtacgtgtcgggcagggggggattagtgaggttcccctcccctctagtgttagcaataatgaaggacactctttgtacaagacgtcaagatgagagcttccacacaggactccacactgtgcttctgtttcaccaggaagaaatcttgaatgtcagccaggcttgtactcatcaattcattcagccagtctctgagggctggtccttctactgagtgctggctagggtggggctgaggactgtgcccctggagagctgccagcctgaggagcaaagccaagtgcgtgtggcccaaagtagacagcatatagggcctgcacgctgaggactgccccaaatgctggcccagctttttccaccagggagggtcagattccaaagccgacagccactcagcacgaggcccagacccaaattccactgccagccacttctactgctgtgctcttcagatgatttatgtctacagtatctgtagagttgaaatactgtataatagtgtgcaattgtgtctcttcccaacatcacattgaagttaactgcttgaaatcagccacagtgggaacacttacaactcagaaatcagcaaatgctataaatcaggcttgatctattcttttgttgtctatctcttgtgggcagagtgtaaatgcactgcagctggacagcctcagagggtgcgggcttcagccagctcctcagtttgatttgtctctgacaatgctggagtgtgctggtctcttgacctcgctgcgccttggtttcc

SEQ ID NO: 14239 - RNA, 333 nt, Homo sapiens
  source 1..333: mol_type = other RNA
gctgggattacaggcatgagccaccgcgcccagcctctaattcttttatttttctttactttttctgattgtattgagataatcaaatgatttttctccttaagggagtatggtaaattgtattaataggtttctaatgtgaaaccagccttacattattggaagaaaacacaatctggtcatgttgcttttaaattatttgctggattcaggttgctaatattttatttaggattttaaaaactcatgtttactagtgatattgactagtaactgcctttccttttttttttttatttccataggtttttggggaacaggtggtatttggtt

SEQ ID NO: 14240 - RNA, 5269 nt, Homo sapiens
  source 1..5269: mol_type = other RNA
gctgggattacaggcatgagccaccgcgcccagcctggaaattctttacagtgtagcactgccccccaaccctgccccataactccgagactgaggggctggatcaaagctggcaagagctctgtccaccatttaataagagcttcagttctgccaagggcattcctaactatttttatactagcatggatgttcgtctcagaggcaaccacagatatgagggtcaggctagattgaggtaaaaaaaaatcctttttgagggcctaggtgcactcatcttggctggctacagcagcaagtaaacatgccagccaactaactacaaagggttcctggaatgagactcttaactacttgccctgggagagaagcaggcccattaaggttcggttaggagaccttgggtttgatttggcagcatctagtcagtttttacctggttcttattttcttctctttagaatgattcaatttcagatgcaactgagacattcatctatacccagtacgtaaataaattaaaggcaaagggacatttccctcacaatagccattggcttatgcagcagggaactcttctttaataaaaatctccttaaatactaacgtcctaagtgtccagtgctgccgcctctgggtacctgaggtgtctgtaactgcagtgggcacctttcacaaatgtgtagctcagtggagactctgatgttagtttcttttattactttgatatatgcgtgctcagctaagttaagcacttatttcacaaagtccttaatctgcttaataaatccttataatatttggtataaaactatttttaaaaattaaattggaagatctttgaattttccattaaatgtttattaataattatccccactggacagcctgaggggtaaagtagatgctctattagttcttctctatcttgtaagttctttttttctagaataataaatataggattcaatgaaagatgaggcacgattcatagtttcctttcctttttactctccttggtttttttgagttaatgggcttttctattgccacaaaaagtcattactaatcatgccgacttaaaaacgtggatcttgagagtacagcttcacatcagagcctctggcagcatggacagcggtgacactttaaaacagtgtccaggagagggtgagcccaggcaaagcttatacaaagaagcctgcagtagacaatataaaccaaacagcataaaaaatgccatacgctatcgcttccaaataaaagctaaatattacagaaacctcacagtgttggaaaaagcaagtttaatttaaaatatagtcactccttccctatcagggtgagccattttttgtctgaatttcctccatgtctcagtgctgcctggcagggcctatgggagagttcatctcaaaagaggtcaacagcaaatgctacagatctgtgtgggaaatgtggctcatcaacattgctaaagctataaccctcattctttagcctggctttccccacttcccactcctccccgaacgcccttccacatctactcccttcaagtgacaactgtacttctacctgaattcaaacattaatatgatatactcagtcaaaagatgagcattcatagtgacaggttgagtgaggctcactgcagtgaccacagcaacaaaagttagggtttgcattcactttcaccagcaaatctaagtgaagaactaagaatgaagtggtgcctgatggggacaagggtttttatctgggcaatttcattctgtttagaaactgacccaatttaaaaaggaagatgtattttactagcactgggggaaaggacggggcactcttgtttttttctctgatggactgagtatggggggtaaagcaacagtagggattatcagatttgggaggaaacaggtcaaggccattggtaatcaactcttcagatatgtacgaggtggactcctaagcagttaacataccctagagaaccaaaagctcccaaaccctgtgaacatgaatgttctagctctccaggagcaagaaagaagctgcaggctaagaagctgcatgccgcactgaagtgagaacgggtgacaggccttcaataagccctggagcatcagctatctctgcccaccctcaattgagttctgagaaaacctaagaatcaatttaaaccaaaccatgtgcttgccctagacctgaaccagggatctgctacagaactgagatagccaggagtgtcctttggctcagcatggaacatgtgctagtctattgcttctttatatgacctgccccttctttagaatgaaggggtattcatgccagtctcagaagtatggaatgattatatgacagcagcaagtagggagggtatgacatatgaaaaccatcccactttgcatggggaaatttgttccatgcatctcactccactcttcagctgctatccccaaaaaaggaagtttgttttaaacccttgaaggttacttcctttgtgggaataaaccctttagacttcatctcccatcttggagccaatcccatccagcaaactgctagcccagggcccctcctcacgtgctctgtccaggactgctcacatccggagggttcttctggtgctgcaaggaggtcctgattagcaggggaatcacatcatggagagaaaacatggctgctctcctgtgtggatatgattgatttacccccccgccccgctttcctccacccagatccctctatattcagaagcaactgatgaaaggatcttcatagaagttacttcttttgtttttaggaaaggagggaactcccaaactcattcaaaagaaagagactataaaatttacgacaggacacgaatcacctggcaccttctactctagacccagcaaggcaaacctagtaatctgttcctgcagtagccttatttcctataagaggaaagatgtatggacaccaatacacaaaagccagtctttgatacatgcctcccattcaggaaaatgtctgtggtctgccttcatcattgttgctggactgcacctgagcttggagatgggtttctgagattcttgcattgccctgcactgttctttgagtgtaaaaaaggatgtaggcctgggttttgcacacttcctcgacactgcatacattcagctttgagtcattgcagtggacccaaaaacctccctctgtgttgtagcaataggctgtgtagtgtcctgagccaaaccctttcccgtgatgcatgaccactgcggagagatcataggcaaaggtctctttgtcaagagaggagagcatgtccctgcagcagtaaggttccatggttaatacctggtcaaagacgacatggaccccaatcttctctcgatgattacggccagaccacctgaatcttttaaggtgcagccggagaacctgaggtagtctgtagatcattaactgctttctagcttcactcagaacaaggggtttgggattggattttcgtcgtttgctgttacactggtcacaagcgtagattctcccttccagggcctctgtctctgtgaatttggccagcatctcagtgagcaagcactctgtttgattcaaagggacaaaccccttttctatgcagtgatagcgttcagggaattccagggataggtcccaaaagggctcaatggtattggatttgtaattgcatgatatacatgtgacctgactgagcagctgcccatgaaatatggtattcaccacctttaagacctgtttggtgagcttcctctgggagaaggggatgaggatccggcgtgtggtgccctcagactcgagttcctgctgcaccttgtgcagcagctcgcagagaaattcctgcgcgtcctgttggtcgtagccgcggaaggcagggatcaggctccacactgagtggagcatggcgaagggcgacactagggcccacttcccggaccacatgactcggaagagggtgtgcagttcacggcagagggaaatgtgctttgaactcggctccttgttctggatgagctccagactccgactaatggaggccctgccgttccagcagaagccctcccgctcgcatgcctcggccctgtcatttctcaaggacagctccgtggccgagctgttggttggcttgccagaaagctgagtcttcccgttggtggctttgggaaacagatgttccgttttggaagggtcaaggttgaggaaacattctcggaacttctggaggtggctgagcacctggaggatggagttcatgtagcaggtgttgcccaggttgcgcaggcccgtgacgcctggggccatggccggctggcgacgcagcttgagtgtggcggcgggcactctgcgtgaggtagggagggcggcggggcgcgaggcagccgggcccgcgtcgcggggcgtgtgcaggagcagccgtgcactcttgcgcggaggggtgctggccagctcctccagcagccgccgtttcacctcgcgccgccgcctccgcgcctcctccttcttgcgctccagggcctcctcctgccgccgctgctccagcttcgcctggccccgggagctcttctcgaaccacagccgcagcgtcctggccagcaggcgctgacgccggtaccacagagccgtgagcatctgcggctgtccctgaggagcgcgctgcggcaggaccacgtcctcacccgaagccatggaccgcagcgtccgcccacgtctcaccggcgtgtcctgtttctggccccggaccgccaggagggagcttcttagcagcttcaggtccccctctgggttatcattgagcacgtagtccttgcacaggtaacagaacacgtagagatcccggacttccatggctagcgggtgtcccgtctcctcaaagtgtttcagggcgtggtcctcaatatagcggccgcaggccacgtgggagcacttgaggcaggcccacacggactcggtggtggcacactctaagcagcaccacttctgagggttcaggatggagtggtcctgggcgagccgtaaccgccctacatgtttgcatctatccatgtcttatagaagtcgccactttctcaacccattaaacaagttttttccatcttcttccatattattccacagtcattggttaggtttcctcttctctattacctggaatgatttaagtgggatattgactggagttgcaggataaactagaggtcctttcaaggtctcttcccatccaaagaatccggtgtgt

SEQ ID NO: 14241 - RNA, 5312 nt, Homo sapiens
  source 1..5312: mol_type = other RNA
gctgggattacaggcatgagccaccgcgcccagcctggaaattctttacagtgtagcactgccccccaaccctgccccataactccgagactgaggggctggatcaaagctggcaagagctctgtccaccatttaataagagcttcagttctgccaagggcattcctaactatttttatactagcatggatgttcgtctcagaggcaaccacagatatgagggtcaggctagattgaggtaaaaaaaaatcctttttgagggcctaggtgcactcatcttggctggctacagcagcaagtaaacatgccagccaactaactacaaagggttcctggaatgagactcttaactacttgccctgggagagaagcaggcccattaaggttcggttaggagaccttgggtttgatttggcagcatctagtcagtttttacctggttcttattttcttctctttagaatgattcaatttcagatgcaactgagacattcatctatacccagtacgtaaataaattaaaggcaaagggacatttccctcacaatagccattggcttatgcagcagggaactcttctttaataaaaatctccttaaatactaacgtcctaagtgtccagtgctgccgcctctgggtacctgaggtgtctgtaactgcagtgggcacctttcacaaatgtgtagctcagtggagactctgatgttagtttcttttattactttgatatatgcgtgctcagctaagttaagcacttatttcacaaagtccttaatctgcttaataaatccttataatatttggtataaaactatttttaaaaattaaattggaagatctttgaattttccattaaatgtttattaataattatccccactggacagcctgaggggtaaagtagatgctctattagttcttctctatcttgtaagttctttttttctagaataataaatataggattcaatgaaagatgaggcacgattcatagtttcctttcctttttactctccttggtttttttgagttaatgggcttttctattgccacaaaaagtcattactaatcatgccgacttaaaaacgtggatcttgagagtacagcttcacatcagagcctctggcagcatggacagcggtgacactttaaaacagtgtccaggagagggtgagcccaggcaaagcttatacaaagaagcctgcagtagacaatataaaccaaacagcataaaaaatgccatacgctatcgcttccaaataaaagctaaatattacagaaacctcacagtgttggaaaaagcaagtttaatttaaaatatagtcactccttccctatcagggtgagccattttttgtctgaatttcctccatgtctcagtgctgcctggcagggcctatgggagagttcatctcaaaagaggtcaacagcaaatgctacagatctgtgtgggaaatgtggctcatcaacattgctaaagctataaccctcattctttagcctggctttccccacttcccactcctccccgaacgcccttccacatctactcccttcaagtgacaactgtacttctacctgaattcaaacattaatatgatatactcagtcaaaagatgagcattcatagtgacaggttgagtgaggctcactgcagtgaccacagcaacaaaagttagggtttgcattcactttcaccagcaaatctaagtgaagaactaagaatgaagtggtgcctgatggggacaagggtttttatctgggcaatttcattctgtttagaaactgacccaatttaaaaaggaagatgtattttactagcactgggggaaaggacggggcactcttgtttttttctctgatggactgagtatggggggtaaagcaacagtagggattatcagatttgggaggaaacaggtcaaggccattggtaatcaactcttcagatatgtacgaggtggactcctaagcagttaacataccctagagaaccaaaagctcccaaaccctgtgaacatgaatgttctagctctccaggagcaagaaagaagctgcaggctaagaagctgcatgccgcactgaagtgagaacgggtgacaggccttcaataagccctggagcatcagctatctctgcccaccctcaattgagttctgagaaaacctaagaatcaatttaaaccaaaccatgtgcttgccctagacctgaaccagggatctgctacagaactgagatagccaggagtgtcctttggctcagcatggaacatgtgctagtctattgcttctttatatgacctgccccttctttagaatgaaggggtattcatgccagtctcagaagtatggaatgattatatgacagcagcaagtagggagggtatgacatatgaaaaccatcccactttgcatggggaaatttgttccatgcatctcactccactcttcagctgctatccccaaaaaaggaagtttgttttaaacccttgaaggttacttcctttgtgggaataaaccctttagacttcatctcccatcttggagccaatcccatccagcaaactgctagcccagggcccctcctcacgtgctctgtccaggactgctcacatccggagggttcttctggtgctgcaaggaggtcctgattagcaggggaatcacatcatggagagaaaacatggctgctctcctgtgtggatatgattgatttacccccccgccccgctttcctccacccagatccctctatattcagaagcaactgatgaaaggatcttcatagaagttacttcttttgtttttaggaaaggagggaactcccaaactcattcaaaagaaagagactataaaatttacgacaggacacgaatcacctggcaccttctactctagacccagcaaggcaaacctagtaatctgttcctgcagtagccttatttcctataagaggaaagatgtatggacaccaatacacaaaagccagtctttgatacatgcctcccattcaggaaaatgtctgtggtctgccttcatcattgttgctggactgcacctgagcttggagatgggtttctgagattcttgcattgccctgcactgttctttgagtgtaaaaaaggatgtaggcctgggttttgcacacttcctcgacactgcatacattcagctttgagtcattgcagtggacccaaaaacctccctctgtgttgtagcaataggctgtgtagtgtcctgagccaaaccctttcccgtgatgcatgaccactgcggagagatcataggcaaaggtctctttgtcaagagaggagagcatgtccctgcagcagtaaggttccatggttaatacctggtcaaagacgacatggaccccaatcttctctcgatgattacggccagaccacctgaatcttttaaggtgcagccggagaacctgaggtagtctgtagatcattaactgctttctagcttcactcagaacaaggggtttgggattggattttcgtcgtttgctgttacactggtcacaagcgtagattctcccttccagggcctctgtctctgtgaatttggccagcatctcagtgagcaagcactctgtttgattcaaagggacaaaccccttttctatgcagtgatagcgttcagggaattccagggataggtcccaaaagggctcaatggtattggatttgtaattgcatgatatacatgtgacctgactgagcagctgcccatgaaatatggtattcaccacctttaagacctgtttggtgagcttcctctgggagaaggggatgaggatccggcgtgtggtgccctcagactcgagttcctgctgcaccttgtgcagcagctcgcagagaaattcctgcgcgtcctgttggtcgtagccgcggaaggcagggatcaggctccacactgagtggagcatggcgaagggcgacactagggcccacttcccggaccacatgactcggaagagggtgtgcagttcacggcagagggaaatgtgctttgaactcggctccttgttctggatgagctccagactccgactaatggaggccctgccgttccagcagaagccctcccgctcgcatgcctcggccctgtcatttctcaaggacagctccgtggccgagctgttggttggcttgccagaaagctgagtcttcccgttggtggctttgggaaacagatgttccgttttggaagggtcaaggttgaggaaacattctcggaacttctggaggtggctgagcacctggaggatggagttcatgtagcaggtgttgcccaggttgcgcaggcccgtgacgcctggggccatggccggctggcgacgcagcttgagtgtggcggcgggcactctgcgtgaggtagggagggcggcggggcgcgaggcagccgggcccgcgtcgcggggcgtgtgcaggagcagccgtgcactcttgcgcggaggggtgctggccagctcctccagcagccgccgtttcacctcgcgccgccgcctccgcgcctcctccttcttgcgctccagggcctcctcctgccgccgctgctccagcttcgcctggccccgggagctcttctcgaaccacagccgcagcgtcctggccagcaggcgctgacgccggtaccacagagccgtgagcatctgcggctgtccctgaggagcgcgctgcggcaggaccacgtcctcacccgaagccatggaccgcagcgtccgcccacgtctcaccggcgtgtcctgtttctggccccggaccgccaggagggagcttcttagcagcttcaggtccccctctgggttatcattgagcacgtagtccttgcacaggtaacagaacacgtagagatcccggacttccatggctagcgggtgtcccgtctcctcaaagtgtttcagggcgtggtcctcaatatagcggccgcaggccacgtgggagcacttgaggcaggcccacacggactcggtggtggcacactctaagcagcaccacttctgagggttcaggatggagtggtcctgggcgagccgtaaccgccctacatgtttgcatctatccatgtcttatagaagtcgccactttctcaacccattaaacaagttttttccatcttcttccatattattccacagtcattggttaggtttcctcttctctattacctggaatgatttaagtgggatattgactggagttgcaggataaactagaggtcctttcaaggtctcttcccatccaaagaatcgccatcatcagcacgcgcgagctgtcaccagggcgcgagacaaccgaacac

SEQ ID NO: 14242 - RNA, 5716 nt, Homo sapiens
  source 1..5716: mol_type = other RNA
gctgggattacaggcatgagccaccgcgcccagcctgtttgattttttgagacagagtctcactcttgtcgcccaggttggagtgcagtggtgcgatctgagctcactgcaacttctgcctcttgggttcaagcgattctcctgcctcagcctcccaagtagctaggactacatacgtccgccaccatgcccagctaattgttgtatttttagtagagacagggtttcaccgtgttggccaggctggtcttgaactccttacctaaggtgatccacctgccccagcttcccaaagtgctgggattacaggagtgagccatggcacctggcctagggttgttatatgtttgacatccgtcccatttgggaggccttctcatcagtcattttatgcctttaatgccattctaggtaggcaggaaaggggtcagggccagtgggcccatgtagcagatagggaaactgaggcccagagaggacaagccacttcttcaagaggacccaaactggatgccaggcaggccctctgcctctgggattttgcccatatggctcaactggcctaagtctgctggcccaaggaaaaatttcaacccaaccctgccctttcccccattcctctcgtgcaggggagttggcgggcctgcggcagcaaataatagctacgcaggagaaagccagtctagacaaggagctgatggcccagaagctggtgcaggctgagcgggaggcccaggcctctctgcgggagcagtgggcagcccaggaggaggacttacagtgactccagcgtgaaaaggttcaggcagctggggaggggtgggcagaagtctgagccagtgtttcatcatcgttcttgctctgcctcggtctgtacatctgtgaaatgggactccctctctgttgtggaggccctggggacagctgggaggactggaggggtggtggggaggttgtggtccttattagacattcagatacccaggtcccaaatctggtccagccctggtaatcctgatgcagagggtccacaaccacatttgggaaatgttgacctaatgcacagcaggaaagcactttcatttgctaagaagtttccatatgaagggccacgcagacctgagcatgtagaaaggcaaggggccagggaagttactagaacactgactctggggttatattgcctgggtttgaatctaatcttggtcgcttactggtgatgctacccaaggtgtctgtgccttcatttccccacctgtagaaatagggataggatagtggaaggtattgaggatgagctgagaccatctgcatagagggcttaacatagtgactggtacttagcaaatgctccatgagttatgattgctggcactggcatgctctccagagtggccctcagaacaggggccctcagccaccaaatcctagacagggcttcctctgacagaggtgcaggctatgactacatggctccagggcatgccactcaccctgcagtccccatggccttgggtggtggttatcacgcttctccatcagggggcggtaaagctctttccgaaagtgctgggattccaggcatgagctatggtgaagctcttaaagaaggggtggcttggccgggcgtgctgactcatgcctgtaatcccagcactttgggaggctgaggtgggcggatcacgaggtcaggagatcgagaccatcctagctaacacagtgaaaccctatctctcctaaaatcacaaaaaattagctgggcatggtggcacgcgcctgtagtcccagatacttgggagggtaaggcagaagaatcgcttcaacctgggaggcagaggttgcagtgagccaaaatcacgccactgcactccagcctgggtgacagagcgagactctgtctaaaaaaaaaaaaaaaaaagaagtggcagctctgtctgcttctcacagagttgctagggacaactgctgaggcaggcacctgccctcgggctccccgggtgggctgctatttgcctgtgggctctgcctgcccgcctgtccagtccccagggatctgaactgtgacctcccccttgctcttcttgccctttgcattgcctggcttggcctcattaatgtccccaaatctgtgttcttctctccagctcctctggcaacccctgacccccttcattcctcacagccagtcctaactctcctccatcccaaccccaatccctcttccacagctgtcggaacatcccctaagctaaaaatcagattgctccttgtcaccttggctcgagtcctctctcccactcccctcactgtccttagaatccccatggcccacacggcctgtcctggcccagccactgcctggggctctggccctgtgactcaccgtgccctgtttccctctgcaccctgcatcctgtagtcctttccaggggctgtgctcttggcctggggtggtcttttctctccttacctggctgacagttacttgtctctccgcaggggatcatgttcggacccccaggccagcccactgctgctccttggcactttcacggccctggcgtgtccccgtcatagcccttatcagtcccttgtatttacctggtcaccctccatctctgagggtatgggggccagatggctcttgctgccctgatgttttggggggtctgcctgggcccctcctggtgtgtcacacgcgtccagtcctggccccctaggaggcagcatggcgggagctggaggccgagcgggcccagctgcagagtcagctgcagcgtgagcaggaggagctgctggcccggcggaaggctgagaaggaacagctgagtgaggagattgctgccctgcagcaggagcatgacgagggcctcctcctggccgagagcgagaagcagcaggttcgtgagccctggcgtggcctctgctgctctctgagctgctccagttctggggccgggccctgctctgccacttggcagctaggagccctggggcaggccactgccctcttgggggcctcagtttccttacctgcaggaggggaggattagaagggggttcgtgaggctttgctgtgctccatgcctggcacacagtgagcacttactgagtgacagtgacagtcgtgacaccaggaaagctgttccatattctcccatgcctcgtcccaccccacgctgggcatggatcctcatggctgccttctgagcagtccccacgatgcccacaggcatcagctgacgtgtccccccaaataacaaatccctaactttcctataatgtaacggagacagggcagactgtgcccatctcctctcctcaccagctgtgtacctgggcgagtcactttacctccttgagcctcagtttcctcatctgtaagatgggtagaaagaaagactctgcagtcagggtgctgtggcgggttagtgagctctatgagtggtatccacgtccgggattcttgtgactgccgttgtgcccttttccagggctgcatgtctgccctgggtccacctgcagtggcacactcaggcctctaagcccccagtgggcacatttcctaggcagcaagaagcctgagcatgcccccaggaccagcccatcccccaagccctttgtcccctgcctctgcccaggccttgtctctgaaggagtctgagaagatggcgctgtcagagaagttgatgggtacacggcacagcctggccaccatctccctggagatggagcggcagaaaccagatgcccagagccggcaggagcaggaccgggtaggcctgccgtcgtagggaggcttgcggagcaggagcgccctctctccaccgagctatcccgcggtttccagcatcccatctggcggactcctcttcctctctcttctcctactctgggtcttctatcctggtgttccttgaatgcctatcttccttttgtgcctcggaacctctcacgcctgccacaagttactcttttccttggtagttctgaactttaaataaggtaatgcctgtaagaatgccataaatgctcaataattgtcatctgttattattttcatcagtaacatcatctgaatcatcagtattgtctgcttttaacagctgcatttttcattgtccaaatatagtcacatacatttgaccattttataattattgaataataaatttgttctgctattttacaatgaaaaataatgctgcagagagcatttttgcacatgtatcgtggcagatgtaggccagaggctcttcttttatccatcctatggccaacctatgaatgtatacacgtttaatgagattttgccagcaatcaaagccttcagggaaaatgtccctagctctttactacatcagatcaaggactctggataattggcataacatcctggaatagctgaaacagagatattattctctgctctcctctgttgtctttgtcttttcacgtcttaataaaagtgctggtgacaagagtgtaactatgtcagtgttctcctgctgtccttgcctgtgtgggtcttctcccaaacccgactttcctccagcggcttcactgaaaaagaggagggggctgtggggggtgggtcggggagcagaggaggaaataaactggatagggaggaagcttctcacaggcccggagagggtaaggaagggagtcaaagacagaattttcttcagcaaacagtaaaaggggaaatctggggatgctaagagtttttaaaccctttgctccatcacataagtaatccatgattttctgttccacaaatcaggactcctactcctccctccctccccatccccaatcctgattcctgtttacaaagaatgttgaaaaacaaggaattatgtataacagttcccagtttgctcaggaaattctcagattataaagagacattacaaatgaacaagtgaagagaagaaccttggtggttccaacatagtatggccattgttttatactcaaaatatagaaagacaacctcagaataagaaaacttttggaatggaataaatcaagtttatcattaaaatgcaaagaaaaaaactctccaaatgttgctgatcttctattttaaactactgttagaccggagaagcggagagcaggggaatccgccaaagagttttggatgaaaattaatcagccctgtctaccgtagtcacaccccactgcccttgagacccaatccttcggaaggagtgtccaagaggtataaagcaaaacgaaaaaacagttcgcaaattccagagttcgttttctctcattaaaaatataaatatcaggctaacacatgttgacacacaataacagggacacagaatccctcctggaagaccgacgggcccacggaccccacgggtgccacggtggtggacgaggttaagtaacttggttcagggtgtctgggcacacctctgcgtgagactctgtctctgctgctcctctcatctctacgccgattcctccccacaatcctcccttttccttgggcccccgacgcctctccgaccaacagtctccccagccccgcagcttctctctttcagacctttacttcttgatcctcactccatagtgagatgtggcctttcagcaaataaattgtgctcagggagactgctcgaacccgttgtgcagaagaggccgccgggtccctttaaggccccgccgcgcctgcgccttgggttatcctgac

SEQ ID NO: 14243 - RNA, 7333 nt, Homo sapiens
  source 1..7333: mol_type = other RNA
gctgggattacaggcatgagccaccgcgcccagctcatcttcttaaaacaaaatccctaggctgtcctccaagccctgagcttggcactcttctctttaaaaattgcactgcactggccaggcacgttggctcacgcctgtgatcccaatgctttgggaggccgaggcagctggatcacttgaggtcaggagtttgagaccagcctgaccaacatggtgaaaccctgtctctactaaaaaatacaaaattagctgggcatggtggtgcatgcctgtaatcccagctacttgggaggctgggaaaggagaatctcttgaacccaggaggcggaggttgcagtgagctgagatcgcaccattgcactccagcctgggcaacagagcgagactctgtctcaaaaaaaaaaaaaagttgcactgcacattcacaaaaagccactctccttggctgcattggagaccctgtatgatctggcctcaggccaccctgacggccctgtttccctctgcccccctcaccccgaccctccagtcctgctccttccaaccccgacacattccatatgtctccgtctcctgaagactcagaccctcctaaggaaaaaggtgcgggtcttggtgatctttttatctaccctggtgcctggcaagcaacaaacaaatatcatcagcagaaagccaggctcagctgagatcatgagagcccaggaagcagttatatcaggagtaacaacctgggtcacagcaggcccaggaccctggaagctgagctcccctatatgggaaaggaagaactaaagccaaacttcaagtgcccttccagagcctgagctcatcactgagaacctctgtctgtcccttctcctgcaaagagaaggacacaggtgggagaggagcatggggtgggaacaaggtcagacataggcctgtggtggtttgatctgttccatacctaggatggggactggagcctgctcagctttcaccttccagcgttacctggagcaaccctgtggggagctgtaggctgtccccatagacttctgagatgtctttctttctctccatctgcaggaagatgtcagagccccagtcttttccctaggagaggcttccctagatggtgggagtcctggcccaggccactgtgggttttacgaagttgaaggtcctggttcggtgatggcacaggggcacacataataacttcctgcctttcagggagcacagctcagctccacagcaggacacctgagcagccagaagctagaaagatgcaagcctgcctccaagtggtcacatgtcataactgcagcccacaacccagaccctccaggcagaggtgcctgggcagcattgactatggcaggccaggcagccaccatcatctggctctgaagattccacgtgctcaggtgaaagagaggtgccggttctacatgagcaaaggagcatcaaagtgtcacacacacatgcattcagactttcaccttttatcatggttttagaaataaggatgcataggccaggtgtggtggttcacgcctgtaatcccagcactttggggggccgaggcaggcagactacctgaggtcaggagttcgagaccagcctagccaacatgacgaaaccccatctctactaaaaatacaaaaaatagccgggcgtggtggcacacgcctgtaatcctagctacttgggaggctgaggcaggagaatcgcttgattcagtggaggttgcagtcagccaagatcacaccattgcactccagcctgggttacaagagcgaaactccgtctccaaaaaaaaaaaaaaaaaaaaaaaaaaaaaaggatgcatgttcagtgaggtcaaataacctactccacttagtttgtaagcatcagtcttgggccaaaagtcatgtccacttgatgctgggattccacttcaatcaaatgaggcaattggactctactgcagctaactgctacttacacatcagaattacccaaggagctttaaacatatttatctatccctctgacccaggctgactgaatcagcatccctgggtgtgggctgggaatgtgtcttttcagcacacttccccagcaagataaaagtgcctctgtaaactgagagcaggaaaccagtgggcaagattgtcaactcatggagtcagggacatgtttaattcatttgtgaatcccctggtactggcacatagaaagcgtcccatattatctgcaaaatgaatgaatgaataaatgagcaagtaggtgaatgaatgattctgaggtctcctccagctttgatggcctatgaccgtgtgactcctgcatatgcatgaacacacagacacagacactacacacatgcacagacacacatacacacttggagcaaagagggatgaagcctgccacactgcaggtggtcctagctgcctgacctcccttcctcacacactgacacacctccctctttgttgacctgttatttattgtgcacccattgggtgcatggcctagccctaggccctggccggagacccaaacatggcctccaagggccaaccttactttgtggaggtgcaagccccagagctggttacaagcatgggaagggaggagggtggcctagcaggaaggctggggaggcagtgtgtcagccggcaggcagcagcgggtagcagaggccccctcttggcgggcagcctacttgcacacttggctgaacagagacaatggtggctggtccctccggcccagcctccttcctacaggcagagccccaagtccatgagtctccggaacctccctcagagaacaagcccagctgggaggcagccagagggcaggatgaggggatttcccaggggagagcagcagagaccctctgagctgccagagatggggaaggggtccaggcaccccacaggaaggaaggtttaaggcatgtgtagaaaggagcacagaaaagtctcccgagcctggcctaggcctcgcctggtcgccagcctccgtcccatccctcacaactctcctgagctgtggctcctgccaggcagacccctaagggaaactgtcgccaccttttacctctctatcctctccagtggtctgaacatagagaacctccttctctgctctgttggaacaaaggctccttgttcctagggttccagggttccctgcaaagctctggaggccccaccccgcccagccctcactcatgccatcagctctgctctgttgatgagcagttgggtatgtgagactgtttcatctacttcgggggaaaggagacacaaggagacaaaggcacagggccccacagccgtgcagagcccttgaagccccccgaggtccctgcccagaaggctgtcccctcagtgggcaggaccttagcgaccctgctccctgggtcacaggaggctggttaggaatttctcaagagtccctgattcactctcctggggcctccccaggaaggtcacctaattcccagagcaagaccatccttggggctgtggctcccctggctgggctgcccaggggcctctgctgccccaagctctcccccagaagccaagggcacaccacataagcactggttctcaaacaagtgctgagttctcagcaagtctaggaaatgaggccactctggattctggggcctggagggtgacatgggctgagctctgggaggaaagtcaagtcctcacctccctcttcccttgggcgtggccagggactggggctgcggagggactgccatgggggtggtggggagcacagcaatattaggaaagcttcagggagcacaagaatgagggccacagggaaacaaggtttgtccttcagcagggaaaggaggtgcctcatccgtcatggtggactcattgaaataagtctcctccagggaggttcatctcaggtctaccctggagcagggaacagtgtctctgaggtggtgctggcttcacagctgattgcggttccgcttagggatgatcttccggtaggttctgcgctctgagatgttgcgcttcaccttggccgtggtgggagcctcatcctggtgcagggacgggctcgagtgggacttcttcaggctgagcttgggctcccgagtgcctccagcttccctccccagctgctcctcccacaggtccagagcatcagaggggcagtgcaggcgggccaccagcagctgcacgtaggtctcgtagcgggttttctcgtactccaggtactccttccgcaggcggtgctcctccagctcgcggccacggccccgccgctccggcaggttcctctgtagatccagcaggtcgtccgcggcagcgtccaggcagttctcgtgggatcgatgctgctcctccagggagctctgggcggggcccacgggcaggatgggccgcacgaatctgcgctgggagcccacagcggcggggaagggcggcgcggagtgcgtggccgcagccaagttgatgcgcgcgatccaggagctcatctccttggcagtgggtgcctggaagaggtagaggcgccagtcagccgtgcgcagctggaagacgtgcggcttcttggtgtaatgcgtggcgggggtggccagcgagtggtgcacccccacgggctcatccaccatctgccccaccaagctctccccctccagacagtggtcttctccctgcttcaggaagtagagaaccatccctcgcagtaaggtgtggaacatcttccagccacgcttgccccatggcgtcttcttgccgtctgcatcttgatgcattttccgagccaggatgccctgcttgtaggtgggcactgtgggatcctgagccagctgaaggaagggcttgctcatcttgccagctggcagggacggctgggccttctcaggtctggctgtgtcttcttcatccacggcccactcgagcttctcgctgcggatagaccagtagagggccttcagcagctccttggggaagttcccgccatccctcagcccattcaggttggttatgaattcctggcagctcatgctcttcccaatgttctgtccatgcaggtccgtgttaagcagcatgattgcacatgtcaaggtgtgtacagaatctactgaggggaagatccccggattgcaatggtggaagcgtctggagaactggtagaggattcgctcccgttcctgagtctccccactgagcaccaaggcctggaggaagctccggagggctcggtccagactctggcctccaaactggaagaaggacaggtactcctcagccacagccctgctaaagtcattgttcttctgcaggtaggcagccacttcagacttccggaagccctccaggcgatagaggcgtgaggccaagttccaggctaccttgttgttcctgacgccattagctagcttgtctccagctggtggtctctggccttcctctggggactgtgcttggggcatagggctcccaggaagccaagaagagttcatcggtgtcctcagattctcatgttctgcagaagtcaggtgaatgtcaggctggacgtctccagtctctgcaggcctggctgttccttcactctttacttcctcgcctggttttggggcctcccctgcctcctttttcttcaaggaacttggctgttccccatccgtctccaagagtgaagactgtgaagcatctagtgtccacttgggcaaaatgcctgagctgtggtgttgaagctgcgggctgccctcctgggacgatgcagggctgggcctgggaccagggcctctgctctcagattctgggctgctaggctctggagaagaagctgggctcctccaggggcagggggccaaggtgcagggaagagattcctgggggtgtccaccctccctctcatctctgtcctgggagttaagagtcacctggggccaaaaaggacctcctctctgccagccctcagggctgagagaggcccaaggttgcacaggatgtgcagcagggccaagatcagatccgacacatcctgattcccaggtcaatgcttcgtccacacacggtgctgcagatggagcaggaccaagcctatctccctcactctccccgtgaccaggaggtgctgcaggagccccctcagcggcagccactgaggcccagcagatggagtgtggtttatagatgggcacagggaatggaggggtacaatgcccactgatagcagcgccgtcccccaaatctggctcactttccagctcccacagcactgtgtcttctgggaggggaggctccagagtcgctgggctctcaggtccagtcctcacacctgcatgggagtctgaagccccccaggaaaagcactctccagaagcactgttctctgagcaaggactcgccaggaagagggggttgctgaagaacatgctctcctcctcagctccccactgtggggaagagtctggggttccctctctcagccatgcctggccctctccctcaggctcactgctgtcttcccctgagtcttcattctcaggtgggctggagtgcaggcccgtgtccccggggaggtccacagggggcgtggggagacagcatttcagcccagccttgagcccttccgtcttctccagctcctcctccaggtctaggacacacatctgggcctgcaggatgcctgcccagaacactacctgtgtggacgtgctccggttctgctttgggctccccggtagatggctgttcactggtgaccctggtgatgctgtgttctgcctgtgctccctctgggcagaggggctccccaggtgtgtgagctccacaccggagccccagggaggagcatcttgtctggtagattcaggagggtcagtggcccgggtttgctcctggcaaggctccagcccgtcctgatggacccagctccccaggtgtgtgagctccacaccggagccccagggaggaacattttgtctggtaggttcaggagggtcagtggcccaggtttgctcctcgaaaggctccggtggatcctcatggctgcacgtttcccttgggcactctcctgggtggggctccaggctgtctcccaagtacaggttgagaatttccatgggctgggggtggtcagggagtctgtagtcacccatcatccactgagcaaaagctgcccaggagtgccccggagcatctgctttcacggtctcactgtgtggactagggggagcactggccgctggagaaactgggaatccatatctaccctccaaaggacccaagaatggatggcttggcctgggctccccaagagcacttcctggctcacagtcggcttgcccagtgaatgt

SEQ ID NO: 14244 - RNA, 6765 nt, Homo sapiens
  source 1..6765: mol_type = other RNA
gctgggattacaggcatgagccaccgcgcccagctgaagatgtggattttttttttttttttttttttgagatggagtctcgcactgtcacccaagctggagtgcagtggcatgatcttggctcactgcaacctccgcctcctgggttcaagtgattctcctgtctcagcctcccaagtagctgggattacaggcgcctgccaccacgcccagctaattttttgtatttttattagagatggggtttcactatgttgccaggctggtctcaaactcctgacctcgtgatccacccgcctcggcctcccaaagtgctgggattacaggcatgtgccaccgcgcctggccagatgtggactctttaaagacatgctctgagtcagaggttcccagccagtgttaggatctctgagagcttacttccttcaatgccccccaggccatggcgtatataatagttacaggagaacagggctggcattcagcaacagggttcaggtacgagctaatgtggacatcagaagtcagcctggcccagaggcagctaggcaggccactaagatacactacataaaccttttcccatggtgttctgggcctaacatgtaatactgcctcttctaactctcacagcctgcttaggttctgcacatagcccagacctgaagcaaagcgcccttgcagagaaaaaaataacagctttaattcacagatttggttggtcttgacctcaagttcttcctttgccacggtctaaatcagggtgtggggctagaggacagataatgagagactgaatcatttatgaaggccttggccaaagagcagctagtgcccactacatggatcccagcagggccaaattctcaacttgttggcttaacaaaagaatgaaaaagctcaaacagaaaacatactggacaaggttggtccagaacatgcaatcctaaatggctatggaataaatttattctgagcaatatctcagtctcacactcactaaattctagggtagttctattgaagatgtttaccatggtttagcgcactgagccctgcacccttccccaggctgccagggaagcagagaggtacaaacattcctaatgccccagtcagcctgttctccctatggggtccctggattacctgcagggacctgggggaaattggctccctgtcttcagctgagagtctggaatctgaaccctagatgaatctactgaagaatgctcaagatgatggataccaagctgagtgagtctaggggagaagagaggcctgaacaaaagagctggggccttcaaagaggtgtatgagaggtgaggttagtagtgccaggctttcctatcttttccttctagtttgctagaaacaagtacaactttagggtgtggggggaaggcaggtagacatgaagaaatggaaatacagttcattctgctagacattttaaactggtttggcttgagaaaaatagaaagtctgtgcctgagaaccttcttttcctctcccttatttaagtacaatagcagctataatctgtgcagttcagctccaaaaaacagggctcctggaagatggctttcatggcagagagttgatggggtagattaatgggctctaggtaaggagcaacaccaagggtccctgaaaactgaggccaacacctgctccctgggggggggccatttgtattccctgacccatgtaacaagcctggccagctgtgggtggaatccatgtggttctatcagaaggctgcagccaacatcaaggccaggcagtcaccagggtcagctgggatctgaagggaggcttctaagaccagacaccctgttagtactaaagatgatgatttgggggtgggatgcctggaggggctggcaccattcaaaaaagtattggaaaacattagccaagaaaaaggctccttgtccctcctaatccatatccagatacccccaaccagagatcttaaaaaggatagaccagccatatgccaacatgccaggattccaaaagcatgcctcaactaattagggtattccctacagcagactggggtagaggggctccatcctggcaataaccagagagccttacctcgcctaggccagggtatggaatctagatgaagactgtccacaaacagtggctctcaagcctgggctaaataaataatattttgcttcattacatggccaaaggagaggaggagatagaaaagatgatattactacctctgtgggctggaagaacttcacctgttggttgaaaggggattaaaggaagataacaggaaaacctggtctggagaagacataaatgaaagctcctggaggccacttttctctgattagaaatctatcctcacactctgcccctagtagactttagcctttggagttcttagggaaaactggctttaagcagcagccagatcaccaaaaacattttccatctggtacaggacccggagctgaagccaaagtagattttggaggaacagctggacaagcaggatgtgtatgtcttacactaagaaactggtccctgtatcagggacttaactcttacttgagatgtacaaagtagatcctactaaattgccctttggaagagaacaatgggcggaggttgggtaggggaaggctttttttttttttttttttttaaactgtaagagaatggttttttaatggaggtagcaggccaagtgaaaaaaagattctgccccctgccttcctgggagattgggagttggcagccatcattcccaagctgatgagtggcatatgactcaccaaggtggtacaacatgggtgggatttttcaaggacaattgccagacctaaaccatcctcctcagaaaatggctttgaagtgggactgcagcactaggagagggcaaattcaagatcaatggccaataataagtacctgaactttaggtctataagcagaagggcatggatttcacctgagccagaaggagatgtgtagcaatagaagcaagaatggcattgtttcagaggaaggaaaagcagagcttggagcaggatgcctctgactaaccacagtggggaggtgggggtggggcagactgtgccttcagctccacagctggtctacaccaacttcctctactcccatccaaacaggtgggctttactatcatatgtaatccacccagaggcacaggcaagccactaaggcaatgcactaccgtaattcaaacagaaagaagaggcatctggattataattgtcacaaggaagggaaaacccaaaccaggtacaaggatcccaaacagggaagatacgcaatagctctaaaaaaaaaaaaaaaaaaagcaggctactaagtttcagtgataatagataataggagaggcagccatgggtgatcagttatgtggacaatggccattgagattgaatttgacaaggcaaactgcttctgagtttcctgatacaagcaggatgttcagcagtaaggacagagtagcagacttcaccaggccctgaggccatccttgctcccttcaggtcctgggacaatcaggccacgctgacctgctttatgaaggttccagagctgaaggttggtcccaggtggtggtccagaatccaagcagagaggaaaaggaccaagctcaggcctcctgagcgaggaagcatccatatctctttttggtcttcctcacagtatcctacttaccgaaatgacagacagttcttcctcttgagaccaattaagattgacctacctaatatatagaatataaaaaaatacagaactttttgacattctctcctttagaagtaaaatatacatgatccaactatggaagaggaagaagaagaagaagaaaggccaaaggcagggatccctgactatcccaatacatgacactctcactccaccctcctctgcaacttacaggtcaccagagcaaggactttctcctcaggagaaaggaaggaccacagccccctatctcaagcttaggagaaaatacagccacctcagaggttctctcaacctcgagggggaattttcaagtaaacaaatgaagttgggtcgcaccatttggaaggtgagtaggaaatatgggatcagtagctacacgtgggaagccccatctgaaggcctgtgctcctcccctgcactcccactggtatacttgagacacttcaggagagtgaggaggatcccccaaactaaagaggtctgggcaaagagtcagagggagggagggacctttgtttcatggtagcctccccagcctctagtcccaggcaatgcaggcagctgggtttactaaaaccaggaacttgtggctcttgggaagagcaatcttaatacaagaaaaatgtgcaaaagaaaaaaaaattaaataactcaatccaagcgtacaagattaatattctgtcagagcaagaacactttgttttggatttctcccttcccctcccacctcccacctctggaatataccgtctgctcaagtacccaagataagagttacacagatcagggcagaggaccgggaagaatgaaaaaagataaagggaaggaagtcaccactgaagaaaaaaagaaaaaaaataaaaataaaaaaaggtgcaaattgattaccttagtcctcctttgtctacccctgggctcctgggttaaagacatgtgtgcagccaaaatatagtgtaaggaagaaaaacccaacacgtccccttcttgtcacaaaacccaaaggtgagcctcagatggttctgtctgtccagagggtgctccctccagggaagggggcggagcaggtcaagagcacagtctccagggcagcagaggtgtgtggtggctgatggtggggacactggtttcccgcccaccagagggctgctcttccgctggctggtggtgcttcccatcccctcccctccctggaggcagatattatagctggaagccctccatgggggcctcaggctgctggaagatgaactgctgttgcgtttcatcgacttggggagccaggctgctatcatcgtcttctacaccaaagtagtgctcaatgaggtcgaaggccttctggtagatctcctggttctcgtggctctggagaaactcaattttatccaagccataggcttcctctatgaggccacaataaggattgacccctgagccactgcgcttgccctcttgctctccaagccgcaggatgttctccagtccattgagggccacttgcacaatcttcgaatccattacagtcagcaagtcacataggggtttgatgcagcccagtgagaccaggtacctgatctgctcaggggttcctcctgatgtggcattggtgatggcccaggctgcctctttccttgtacgaaactctgctttctgaaggatttcgatcaacacagggaagatatttgcatctataacagcctgtatttgagccctgttgccagcagtaatatttgaaatagtccagcaagcttccttccggattgactccttgggactgctcaacaagtggagaaggcaaggtagggctgaacagttaagaatgacctgggtctggatgtcatccccagtgacgatgttacccacggctctcagggcaggagaagccactttgtaatcattgtgcatcagcagctctaccaatctccggcagactccggagtctatgactgcctggatcttctcattggggccatcagacagataagaaagggcccagcaagcatctgccagcaagtccgagtcgctgctgaagagtaggcgagacagtacaggcaaacaaggagagacctttgcaaactctgggggtgggtttttccctcggcagagatttgacagggcccagactgcattccgtgtcatcgtcagtcgtgtggacttggtaaggagtgttaacaaaggattaaggatggaacagttcaagacgtaatctcggcaaacagagctatctccagctatgtttcccagtgcccagactgcctgttcctgaacatcctcaaagtctgaattaagcagctctataaaaatggggacagcccctgcttcaatgacaattttggtctgctgagaggttccagaggcaatattcgttagagcccaggcagcttcaaactgtaatgtacaattctcattcctcttcagaaactccacgaaccgatccaccactcttggagtgttgataacttcatctattggaggactaggctctttggagagcagtttccggaatttctgtgtggttgctaactgcaggtcagaatcatcagaaaagagcatctccaccatctctcttgtgatcacactctccccagtggtagagctcacataagagtccatgagaagactatcgaacatggcagcttcttcattaatcagctccacatttctccgtttaaaaagttgttgctctcgcttctgcttccggagctgaatgccctcttcctctcttcttcgtctcatttcttcagggtttagagcattgttcttatagctcttcattcgataattgtctttccctgggctcgccatggtctcatccagattcaatgatcaactagcagccattcatatctatgcttctgcctctcccagatccttgaagcaaattcctgacctatcacttcatccacatttcagtatgtatccatcgcgggtccgctcgctcactcttggcggcggaggcaacggcggcagcttcagcggcagctttcagtagacaatatggcggatctgtag

SEQ ID NO: 14245 - RNA, 6642 nt, Homo sapiens
  source 1..6642: mol_type = other RNA
gctgggattacaggcatgagccaccgcgcccagctgaagatgtggattttttttttttttttttttttgagatggagtctcgcactgtcacccaagctggagtgcagtggcatgatcttggctcactgcaacctccgcctcctgggttcaagtgattctcctgtctcagcctcccaagtagctgggattacaggcgcctgccaccacgcccagctaattttttgtatttttattagagatggggtttcactatgttgccaggctggtctcaaactcctgacctcgtgatccacccgcctcggcctcccaaagtgctgggattacaggcatgtgccaccgcgcctggccagatgtggactctttaaagacatgctctgagtcagaggttcccagccagtgttaggatctctgagagcttacttccttcaatgccccccaggccatggcgtatataatagttacaggagaacagggctggcattcagcaacagggttcaggtacgagctaatgtggacatcagaagtcagcctggcccagaggcagctaggcaggccactaagatacactacataaaccttttcccatggtgttctgggcctaacatgtaatactgcctcttctaactctcacagcctgcttaggttctgcacatagcccagacctgaagcaaagcgcccttgcagagaaaaaaataacagctttaattcacagatttggttggtcttgacctcaagttcttcctttgccacggtctaaatcagggtgtggggctagaggacagataatgagagactgaatcatttatgaaggccttggccaaagagcagctagtgcccactacatggatcccagcagggccaaattctcaacttgttggcttaacaaaagaatgaaaaagctcaaacagaaaacatactggacaaggttggtccagaacatgcaatcctaaatggctatggaataaatttattctgagcaatatctcagtctcacactcactaaattctagggtagttctattgaagatgtttaccatggtttagcgcactgagccctgcacccttccccaggctgccagggaagcagagaggtacaaacattcctaatgccccagtcagcctgttctccctatggggtccctggattacctgcagggacctgggggaaattggctccctgtcttcagctgagagtctggaatctgaaccctagatgaatctactgaagaatgctcaagatgatggataccaagctgagtgagtctaggggagaagagaggcctgaacaaaagagctggggccttcaaagaggtgtatgagaggtgaggttagtagtgccaggctttcctatcttttccttctagtttgctagaaacaagtacaactttagggtgtggggggaaggcaggtagacatgaagaaatggaaatacagttcattctgctagacattttaaactggtttggcttgagaaaaatagaaagtctgtgcctgagaaccttcttttcctctcccttatttaagtacaatagcagctataatctgtgcagttcagctccaaaaaacagggctcctggaagatggctttcatggcagagagttgatggggtagattaatgggctctaggtaaggagcaacaccaagggtccctgaaaactgaggccaacacctgctccctgggggggggccatttgtattccctgacccatgtaacaagcctggccagctgtgggtggaatccatgtggttctatcagaaggctgcagccaacatcaaggccaggcagtcaccagggtcagctgggatctgaagggaggcttctaagaccagacaccctgttagtactaaagatgatgatttgggggtgggatgcctggaggggctggcaccattcaaaaaagtattggaaaacattagccaagaaaaaggctccttgtccctcctaatccatatccagatacccccaaccagagatcttaaaaaggatagaccagccatatgccaacatgccaggattccaaaagcatgcctcaactaattagggtattccctacagcagactggggtagaggggctccatcctggcaataaccagagagccttacctcgcctaggccagggtatggaatctagatgaagactgtccacaaacagtggctctcaagcctgggctaaataaataatattttgcttcattacatggccaaaggagaggaggagatagaaaagatgatattactacctctgtgggctggaagaacttcacctgttggttgaaaggggattaaaggaagataacaggaaaacctggtctggagaagacataaatgaaagctcctggaggccacttttctctgattagaaatctatcctcacactctgcccctagtagactttagcctttggagttcttagggaaaactggctttaagcagcagccagatcaccaaaaacattttccatctggtacaggacccggagctgaagccaaagtagattttggaggaacagctggacaagcaggatgtgtatgtcttacactaagaaactggtccctgtatcagggacttaactcttacttgagatgtacaaagtagatcctactaaattgccctttggaagagaacaatgggcggaggttgggtaggggaaggctttttttttttttttttttttaaactgtaagagaatggttttttaatggaggtagcaggccaagtgaaaaaaagattctgccccctgccttcctgggagattgggagttggcagccatcattcccaagctgatgagtggcatatgactcaccaaggtggtacaacatgggtgggatttttcaaggacaattgccagacctaaaccatcctcctcagaaaatggctttgaagtgggactgcagcactaggagagggcaaattcaagatcaatggccaataataagtacctgaactttaggtctataagcagaagggcatggatttcacctgagccagaaggagatgtgtagcaatagaagcaagaatggcattgtttcagaggaaggaaaagcagagcttggagcaggatgcctctgactaaccacagtggggaggtgggggtggggcagactgtgccttcagctccacagctggtctacaccaacttcctctactcccatccaaacaggtgggctttactatcatatgtaatccacccagaggcacaggcaagccactaaggcaatgcactaccgtaattcaaacagaaagaagaggcatctggattataattgtcacaaggaagggaaaacccaaaccaggtacaaggatcccaaacagggaagatacgcaatagctctaaaaaaaaaaaaaaaaaaagcaggctactaagtttcagtgataatagataataggagaggcagccatgggtgatcagttatgtggacaatggccattgagattgaatttgacaaggcaaactgcttctgagtttcctgatacaagcaggatgttcagcagtaaggacagagtagcagacttcaccaggccctgaggccatccttgctcccttcaggtcctgggacaatcaggccacgctgacctgctttatgaaggttccagagctgaaggttggtcccaggtggtggtccagaatccaagcagagaggaaaaggaccaagctcaggcctcctgagcgaggaagcatccatatctctttttggtcttcctcacagtatcctacttaccgaaatgacagacagttcttcctcttgagaccaattaagattgacctacctaatatatagaatataaaaaaatacagaactttttgacattctctcctttagaagtaaaatatacatgatccaactatggaagaggaagaagaagaagaagaaaggccaaaggcagggatccctgactatcccaatacatgacactctcactccaccctcctctgcaacttacaggtcaccagagcaaggactttctcctcaggagaaaggaaggaccacagccccctatctcaagcttaggagaaaatacagccacctcagaggttctctcaacctcgagggggaattttcaagtaaacaaatgaagttgggtcgcaccatttggaaggtgagtaggaaatatgggatcagtagctacacgtgggaagccccatctgaaggcctgtgctcctcccctgcactcccactggtatacttgagacacttcaggagagtgaggaggatcccccaaactaaagaggtctgggcaaagagtcagagggagggagggacctttgtttcatggtagcctccccagcctctagtcccaggcaatgcaggcagctgggtttactaaaaccaggaacttgtggctcttgggaagagcaatcttaatacaagaaaaatgtgcaaaagaaaaaaaaattaaataactcaatccaagcgtacaagattaatattctgtcagagcaagaacactttgttttggatttctcccttcccctcccacctcccacctctggaatataccgtctgctcaagtacccaagataagagttacacagatcagggcagaggaccgggaagaatgaaaaaagataaagggaaggaagtcaccactgaagaaaaaaagaaaaaaaataaaaataaaaaaaggtgcaaattgattaccttagtcctcctttgtctacccctgggctcctgggttaaagacatgtgtgcagccaaaatatagtgtaaggaagaaaaacccaacacgtccccttcttgtcacaaaacccaaaggtgagcctcagatggttctgtctgtccagagggtgctccctccagggaagggggcggagcaggtcaagagcacagtctccagggcagcagaggtgtgtggtggctgatggtggggacactggtttcccgcccaccagagggctgctcttccgctggctggtggtgcttcccatcccctcccctccctggaggcagatattatagctggaagccctccatgggggcctcaggctgctggaagatgaactgctgttgcgtttcatcgacttggggagccaggctgctatcatcgtcttctacaccaaagtagtgctcaatgaggtcgaaggccttctggtagatctcctggttctcgtggctctggagaaactcaattttatccaagccataggcttcctctatgaggccacaataaggattgacccctgagccactgcgcttgccctcttgctctccaagccgcaggatgttctccagtccattgagggccacttgcacaatcttcgaatccattacagtcagcaagtcacataggggtttgatgcagcccagtgagaccaggtacctgatctgctcaggggttcctcctgatgtggcattggtgatggcccaggctgcctctttccttgtacgaaactctgctttctgaaggatttcgatcaacacagggaagatatttgcatctataacagcctgtatttgagccctgttgccagcagtaatatttgaaatagtccagcaagcttccttccggattgactccttgggactgctcaacaagtggagaaggcaaggtagggctgaacagttaagaatgacctgggtctggatgtcatccccagtgacgatgttacccacggctctcagggcaggagaagccactttgtaatcattgtgcatcagcagctctaccaatctccggcagactccggagtctatgactgcctggatcttctcattggggccatcagacagataagaaagggcccagcaagcatctgccagcaagtccgagtcgctgctgaagagtaggcgagacagtacaggcaaacaaggagagacctttgcaaactctgggggtgggtttttccctcggcagagatttgacagggcccagactgcattccgtgtcatcgtcagtcgtgtggacttggtaaggagtgttaacaaaggattaaggatggaacagttcaagacgtaatctcggcaaacagagctatctccagctatgtttcccagtgcccagactgcctgttcctgaacatcctcaaagtctgaattaagcagctctataaaaatggggacagcccctgcttcaatgacaattttggtctgctgagaggttccagaggcaatattcgttagagcccaggcagcttcaaactgtaatgtacaattctcattcctcttcagaaactccacgaaccgatccaccactcttggagtgttgataacttcatctattggaggactaggctctttggagagcagtttccggaatttctgtgtggttgctaactgcaggtcagaatcatcagaaaagagcatctccaccatctctcttgtgatcacactctccccagtggtagagctcacataagagtccatgagaagactatcgaacatggcagcttcttcattaatcagctccacatttctccgtttaaaaagttgttgctctcgcttctgcttccggagctgaatgccctcttcctctcttcttcgtctcatttcttcagggtttagagcattgttcttatagctcttcattcgataattgtctttccctgggctcgccatggtctccatcgcgggtccgctcgctcactcttggcggcggaggcaacggcggcagcttcagcggcagctttcagtagacaatat

SEQ ID NO: 14246 - RNA, 6973 nt, Homo sapiens
  source 1..6973: mol_type = other RNA
gctgggattacaggcatgagccaccgcgcccagctgaagatgtggattttttttttttttttttttttgagatggagtctcgcactgtcacccaagctggagtgcagtggcatgatcttggctcactgcaacctccgcctcctgggttcaagtgattctcctgtctcagcctcccaagtagctgggattacaggcgcctgccaccacgcccagctaattttttgtatttttattagagatggggtttcactatgttgccaggctggtctcaaactcctgacctcgtgatccacccgcctcggcctcccaaagtgctgggattacaggcatgtgccaccgcgcctggccagatgtggactctttaaagacatgctctgagtcagaggttcccagccagtgttaggatctctgagagcttacttccttcaatgccccccaggccatggcgtatataatagttacaggagaacagggctggcattcagcaacagggttcaggtacgagctaatgtggacatcagaagtcagcctggcccagaggcagctaggcaggccactaagatacactacataaaccttttcccatggtgttctgggcctaacatgtaatactgcctcttctaactctcacagcctgcttaggttctgcacatagcccagacctgaagcaaagcgcccttgcagagaaaaaaataacagctttaattcacagatttggttggtcttgacctcaagttcttcctttgccacggtctaaatcagggtgtggggctagaggacagataatgagagactgaatcatttatgaaggccttggccaaagagcagctagtgcccactacatggatcccagcagggccaaattctcaacttgttggcttaacaaaagaatgaaaaagctcaaacagaaaacatactggacaaggttggtccagaacatgcaatcctaaatggctatggaataaatttattctgagcaatatctcagtctcacactcactaaattctagggtagttctattgaagatgtttaccatggtttagcgcactgagccctgcacccttccccaggctgccagggaagcagagaggtacaaacattcctaatgccccagtcagcctgttctccctatggggtccctggattacctgcagggacctgggggaaattggctccctgtcttcagctgagagtctggaatctgaaccctagatgaatctactgaagaatgctcaagatgatggataccaagctgagtgagtctaggggagaagagaggcctgaacaaaagagctggggccttcaaagaggtgtatgagaggtgaggttagtagtgccaggctttcctatcttttccttctagtttgctagaaacaagtacaactttagggtgtggggggaaggcaggtagacatgaagaaatggaaatacagttcattctgctagacattttaaactggtttggcttgagaaaaatagaaagtctgtgcctgagaaccttcttttcctctcccttatttaagtacaatagcagctataatctgtgcagttcagctccaaaaaacagggctcctggaagatggctttcatggcagagagttgatggggtagattaatgggctctaggtaaggagcaacaccaagggtccctgaaaactgaggccaacacctgctccctgggggggggccatttgtattccctgacccatgtaacaagcctggccagctgtgggtggaatccatgtggttctatcagaaggctgcagccaacatcaaggccaggcagtcaccagggtcagctgggatctgaagggaggcttctaagaccagacaccctgttagtactaaagatgatgatttgggggtgggatgcctggaggggctggcaccattcaaaaaagtattggaaaacattagccaagaaaaaggctccttgtccctcctaatccatatccagatacccccaaccagagatcttaaaaaggatagaccagccatatgccaacatgccaggattccaaaagcatgcctcaactaattagggtattccctacagcagactggggtagaggggctccatcctggcaataaccagagagccttacctcgcctaggccagggtatggaatctagatgaagactgtccacaaacagtggctctcaagcctgggctaaataaataatattttgcttcattacatggccaaaggagaggaggagatagaaaagatgatattactacctctgtgggctggaagaacttcacctgttggttgaaaggggattaaaggaagataacaggaaaacctggtctggagaagacataaatgaaagctcctggaggccacttttctctgattagaaatctatcctcacactctgcccctagtagactttagcctttggagttcttagggaaaactggctttaagcagcagccagatcaccaaaaacattttccatctggtacaggacccggagctgaagccaaagtagattttggaggaacagctggacaagcaggatgtgtatgtcttacactaagaaactggtccctgtatcagggacttaactcttacttgagatgtacaaagtagatcctactaaattgccctttggaagagaacaatgggcggaggttgggtaggggaaggctttttttttttttttttttttaaactgtaagagaatggttttttaatggaggtagcaggccaagtgaaaaaaagattctgccccctgccttcctgggagattgggagttggcagccatcattcccaagctgatgagtggcatatgactcaccaaggtggtacaacatgggtgggatttttcaaggacaattgccagacctaaaccatcctcctcagaaaatggctttgaagtgggactgcagcactaggagagggcaaattcaagatcaatggccaataataagtacctgaactttaggtctataagcagaagggcatggatttcacctgagccagaaggagatgtgtagcaatagaagcaagaatggcattgtttcagaggaaggaaaagcagagcttggagcaggatgcctctgactaaccacagtggggaggtgggggtggggcagactgtgccttcagctccacagctggtctacaccaacttcctctactcccatccaaacaggtgggctttactatcatatgtaatccacccagaggcacaggcaagccactaaggcaatgcactaccgtaattcaaacagaaagaagaggcatctggattataattgtcacaaggaagggaaaacccaaaccaggtacaaggatcccaaacagggaagatacgcaatagctctaaaaaaaaaaaaaaaaaaagcaggctactaagtttcagtgataatagataataggagaggcagccatgggtgatcagttatgtggacaatggccattgagattgaatttgacaaggcaaactgcttctgagtttcctgatacaagcaggatgttcagcagtaaggacagagtagcagacttcaccaggccctgaggccatccttgctcccttcaggtcctgggacaatcaggccacgctgacctgctttatgaaggttccagagctgaaggttggtcccaggtggtggtccagaatccaagcagagaggaaaaggaccaagctcaggcctcctgagcgaggaagcatccatatctctttttggtcttcctcacagtatcctacttaccgaaatgacagacagttcttcctcttgagaccaattaagattgacctacctaatatatagaatataaaaaaatacagaactttttgacattctctcctttagaagtaaaatatacatgatccaactatggaagaggaagaagaagaagaagaaaggccaaaggcagggatccctgactatcccaatacatgacactctcactccaccctcctctgcaacttacaggtcaccagagcaaggactttctcctcaggagaaaggaaggaccacagccccctatctcaagcttaggagaaaatacagccacctcagaggttctctcaacctcgagggggaattttcaagtaaacaaatgaagttgggtcgcaccatttggaaggtgagtaggaaatatgggatcagtagctacacgtgggaagccccatctgaaggcctgtgctcctcccctgcactcccactggtatacttgagacacttcaggagagtgaggaggatcccccaaactaaagaggtctgggcaaagagtcagagggagggagggacctttgtttcatggtagcctccccagcctctagtcccaggcaatgcaggcagctgggtttactaaaaccaggaacttgtggctcttgggaagagcaatcttaatacaagaaaaatgtgcaaaagaaaaaaaaattaaataactcaatccaagcgtacaagattaatattctgtcagagcaagaacactttgttttggatttctcccttcccctcccacctcccacctctggaatataccgtctgctcaagtacccaagataagagttacacagatcagggcagaggaccgggaagaatgaaaaaagataaagggaaggaagtcaccactgaagaaaaaaagaaaaaaaataaaaataaaaaaaggtgcaaattgattaccttagtcctcctttgtctacccctgggctcctgggttaaagacatgtgtgcagccaaaatatagtgtaaggaagaaaaacccaacacgtccccttcttgtcacaaaacccaaaggtgagcctcagatggttctgtctgtccagagggtgctccctccagggaagggggcggagcaggtcaagagcacagtctccagggcagcagaggtgtgtggtggctgatggtggggacactggtttcccgcccaccagagggctgctcttccgctggctggtggtgcttcccatcccctcccctccctggaggcagatattatagctggaagccctccatgggggcctcaggctgctggaagatgaactgctgttgcgtttcatcgacttggggagccaggctgctatcatcgtcttctacaccaaagtagtgctcaatgaggtcgaaggccttctggtagatctcctggttctcgtggctctggagaaactcaattttatccaagccataggcttcctctatgaggccacaataaggattgacccctgagccactgcgcttgccctcttgctctccaagccgcaggatgttctccagtccattgagggccacttgcacaatcttcgaatccattacagtcagcaagtcacataggggtttgatgcagcccagtgagaccaggtacctgatctgctcaggggttcctcctgatgtggcattggtgatggcccaggctgcctctttccttgtacgaaactctgctttctgaaggatttcgatcaacacagggaagatatttgcatctataacagcctgtatttgagccctgttgccagcagtaatatttgaaatagtccagcaagcttccttccggattgactccttgggactgctcaacaagtggagaaggcaaggtagggctgaacagttaagaatgacctgggtctggatgtcatccccagtgacgatgttacccacggctctcagggcaggagaagccactttgtaatcattgtgcatcagcagctctaccaatctccggcagactccggagtctatgactgcctggatcttctcattggggccatcagacagataagaaagggcccagcaagcatctgccagcaagtccgagtcgctgctgaagagtaggcgagacagtacaggcaaacaaggagagacctttgcaaactctgggggtgggtttttccctcggcagagatttgacagggcccagactgcattccgtgtcatcgtcagtcgtgtggacttggtaaggagtgttaacaaaggattaaggatggaacagttcaagacgtaatctcggcaaacagagctatctccagctatgtttcccagtgcccagactgcctgttcctgaacatcctcaaagtctgaattaagcagctctataaaaatggggacagcccctgcttcaatgacaattttggtctgctgagaggttccagaggcaatattcgttagagcccaggcagcttcaaactgtaatgtacaattctcattcctcttcagaaactccacgaaccgatccaccactcttggagtgttgataacttcatctattggaggactaggctctttggagagcagtttccggaatttctgtgtggttgctaactgcaggtcagaatcatcagaaaagagcatctccaccatctctcttgtgatcacactctccccagtggtagagctcacataagagtccatgagaagactatcgaacatggcagcttcttcattaatcagctccacatttctccgtttaaaaagttgttgctctcgcttctgcttccggagctgaatgccctcttcctctcttcttcgtctcatttcttcagggtttagagcattgttcttatagctcttcattcgataattgtctttccctgggctcgccatggtctcggcctagtgctggctcgcctgacgtcccctcactagaggactccacctcgctacgtaggtaggacttccctgagttcaggggagccactgaatctagtcaagacacgcgttggccaaacacaacccaggagaaagctaccttagcgccgcccaggcctgccgccgggagcccgtcccccagccccagtctgggcgcaggacagagagtaggcccctttctacctcccaggaacacgtgggctcctgcccgaggccaccatgtggggggctccaggcgtgccaaggtgtccccgaaaccagcaccaaaggactgcttccagcacgggccctagctcggcccaaaactggcaagaggggcactcccggcctgacttttcccctcagacctagctagaggggatgcagacat

SEQ ID NO: 14247 - RNA, 7016 nt, Homo sapiens
  source 1..7016: mol_type = other RNA
gctgggattacaggcatgagccaccgcgcccagctgaagatgtggattttttttttttttttttttttgagatggagtctcgcactgtcacccaagctggagtgcagtggcatgatcttggctcactgcaacctccgcctcctgggttcaagtgattctcctgtctcagcctcccaagtagctgggattacaggcgcctgccaccacgcccagctaattttttgtatttttattagagatggggtttcactatgttgccaggctggtctcaaactcctgacctcgtgatccacccgcctcggcctcccaaagtgctgggattacaggcatgtgccaccgcgcctggccagatgtggactctttaaagacatgctctgagtcagaggttcccagccagtgttaggatctctgagagcttacttccttcaatgccccccaggccatggcgtatataatagttacaggagaacagggctggcattcagcaacagggttcaggtacgagctaatgtggacatcagaagtcagcctggcccagaggcagctaggcaggccactaagatacactacataaaccttttcccatggtgttctgggcctaacatgtaatactgcctcttctaactctcacagcctgcttaggttctgcacatagcccagacctgaagcaaagcgcccttgcagagaaaaaaataacagctttaattcacagatttggttggtcttgacctcaagttcttcctttgccacggtctaaatcagggtgtggggctagaggacagataatgagagactgaatcatttatgaaggccttggccaaagagcagctagtgcccactacatggatcccagcagggccaaattctcaacttgttggcttaacaaaagaatgaaaaagctcaaacagaaaacatactggacaaggttggtccagaacatgcaatcctaaatggctatggaataaatttattctgagcaatatctcagtctcacactcactaaattctagggtagttctattgaagatgtttaccatggtttagcgcactgagccctgcacccttccccaggctgccagggaagcagagaggtacaaacattcctaatgccccagtcagcctgttctccctatggggtccctggattacctgcagggacctgggggaaattggctccctgtcttcagctgagagtctggaatctgaaccctagatgaatctactgaagaatgctcaagatgatggataccaagctgagtgagtctaggggagaagagaggcctgaacaaaagagctggggccttcaaagaggtgtatgagaggtgaggttagtagtgccaggctttcctatcttttccttctagtttgctagaaacaagtacaactttagggtgtggggggaaggcaggtagacatgaagaaatggaaatacagttcattctgctagacattttaaactggtttggcttgagaaaaatagaaagtctgtgcctgagaaccttcttttcctctcccttatttaagtacaatagcagctataatctgtgcagttcagctccaaaaaacagggctcctggaagatggctttcatggcagagagttgatggggtagattaatgggctctaggtaaggagcaacaccaagggtccctgaaaactgaggccaacacctgctccctgggggggggccatttgtattccctgacccatgtaacaagcctggccagctgtgggtggaatccatgtggttctatcagaaggctgcagccaacatcaaggccaggcagtcaccagggtcagctgggatctgaagggaggcttctaagaccagacaccctgttagtactaaagatgatgatttgggggtgggatgcctggaggggctggcaccattcaaaaaagtattggaaaacattagccaagaaaaaggctccttgtccctcctaatccatatccagatacccccaaccagagatcttaaaaaggatagaccagccatatgccaacatgccaggattccaaaagcatgcctcaactaattagggtattccctacagcagactggggtagaggggctccatcctggcaataaccagagagccttacctcgcctaggccagggtatggaatctagatgaagactgtccacaaacagtggctctcaagcctgggctaaataaataatattttgcttcattacatggccaaaggagaggaggagatagaaaagatgatattactacctctgtgggctggaagaacttcacctgttggttgaaaggggattaaaggaagataacaggaaaacctggtctggagaagacataaatgaaagctcctggaggccacttttctctgattagaaatctatcctcacactctgcccctagtagactttagcctttggagttcttagggaaaactggctttaagcagcagccagatcaccaaaaacattttccatctggtacaggacccggagctgaagccaaagtagattttggaggaacagctggacaagcaggatgtgtatgtcttacactaagaaactggtccctgtatcagggacttaactcttacttgagatgtacaaagtagatcctactaaattgccctttggaagagaacaatgggcggaggttgggtaggggaaggctttttttttttttttttttttaaactgtaagagaatggttttttaatggaggtagcaggccaagtgaaaaaaagattctgccccctgccttcctgggagattgggagttggcagccatcattcccaagctgatgagtggcatatgactcaccaaggtggtacaacatgggtgggatttttcaaggacaattgccagacctaaaccatcctcctcagaaaatggctttgaagtgggactgcagcactaggagagggcaaattcaagatcaatggccaataataagtacctgaactttaggtctataagcagaagggcatggatttcacctgagccagaaggagatgtgtagcaatagaagcaagaatggcattgtttcagaggaaggaaaagcagagcttggagcaggatgcctctgactaaccacagtggggaggtgggggtggggcagactgtgccttcagctccacagctggtctacaccaacttcctctactcccatccaaacaggtgggctttactatcatatgtaatccacccagaggcacaggcaagccactaaggcaatgcactaccgtaattcaaacagaaagaagaggcatctggattataattgtcacaaggaagggaaaacccaaaccaggtacaaggatcccaaacagggaagatacgcaatagctctaaaaaaaaaaaaaaaaaaagcaggctactaagtttcagtgataatagataataggagaggcagccatgggtgatcagttatgtggacaatggccattgagattgaatttgacaaggcaaactgcttctgagtttcctgatacaagcaggatgttcagcagtaaggacagagtagcagacttcaccaggccctgaggccatccttgctcccttcaggtcctgggacaatcaggccacgctgacctgctttatgaaggttccagagctgaaggttggtcccaggtggtggtccagaatccaagcagagaggaaaaggaccaagctcaggcctcctgagcgaggaagcatccatatctctttttggtcttcctcacagtatcctacttaccgaaatgacagacagttcttcctcttgagaccaattaagattgacctacctaatatatagaatataaaaaaatacagaactttttgacattctctcctttagaagtaaaatatacatgatccaactatggaagaggaagaagaagaagaagaaaggccaaaggcagggatccctgactatcccaatacatgacactctcactccaccctcctctgcaacttacaggtcaccagagcaaggactttctcctcaggagaaaggaaggaccacagccccctatctcaagcttaggagaaaatacagccacctcagaggttctctcaacctcgagggggaattttcaagtaaacaaatgaagttgggtcgcaccatttggaaggtgagtaggaaatatgggatcagtagctacacgtgggaagccccatctgaaggcctgtgctcctcccctgcactcccactggtatacttgagacacttcaggagagtgaggaggatcccccaaactaaagaggtctgggcaaagagtcagagggagggagggacctttgtttcatggtagcctccccagcctctagtcccaggcaatgcaggcagctgggtttactaaaaccaggaacttgtggctcttgggaagagcaatcttaatacaagaaaaatgtgcaaaagaaaaaaaaattaaataactcaatccaagcgtacaagattaatattctgtcagagcaagaacactttgttttggatttctcccttcccctcccacctcccacctctggaatataccgtctgctcaagtacccaagataagagttacacagatcagggcagaggaccgggaagaatgaaaaaagataaagggaaggaagtcaccactgaagaaaaaaagaaaaaaaataaaaataaaaaaaggtgcaaattgattaccttagtcctcctttgtctacccctgggctcctgggttaaagacatgtgtgcagccaaaatatagtgtaaggaagaaaaacccaacacgtccccttcttgtcacaaaacccaaaggtgagcctcagatggttctgtctgtccagagggtgctccctccagggaagggggcggagcaggtcaagagcacagtctccagggcagcagaggtgtgtggtggctgatggtggggacactggtttcccgcccaccagagggctgctcttccgctggctggtggtgcttcccatcccctcccctccctggaggcagatattatagctggaagccctccatgggggcctcaggctgctggaagatgaactgctgttgcgtttcatcgacttggggagccaggctgctatcatcgtcttctacaccaaagtagtgctcaatgaggtcgaaggccttctggtagatctcctggttctcgtggctctggagaaactcaattttatccaagccataggcttcctctatgaggccacaataaggattgacccctgagccactgcgcttgccctcttgctctccaagccgcaggatgttctccagtccattgagggccacttgcacaatcttcgaatccattacagtcagcaagtcacataggggtttgatgcagcccagtgagaccaggtacctgatctgctcaggggttcctcctgatgtggcattggtgatggcccaggctgcctctttccttgtacgaaactctgctttctgaaggatttcgatcaacacagggaagatatttgcatctataacagcctgtatttgagccctgttgccagcagtaatatttgaaatagtccagcaagcttccttccggattgactccttgggactgctcaacaagtggagaaggcaaggtagggctgaacagttaagaatgacctgggtctggatgtcatccccagtgacgatgttacccacggctctcagggcaggagaagccactttgtaatcattgtgcatcagcagctctaccaatctccggcagactccggagtctatgactgcctggatcttctcattggggccatcagacagataagaaagggcccagcaagcatctgccagcaagtccgagtcgctgctgaagagtaggcgagacagtacaggcaaacaaggagagacctttgcaaactctgggggtgggtttttccctcggcagagatttgacagggcccagactgcattccgtgtcatcgtcagtcgtgtggacttggtaaggagtgttaacaaaggattaaggatggaacagttcaagacgtaatctcggcaaacagagctatctccagctatgtttcccagtgcccagactgcctgttcctgaacatcctcaaagtctgaattaagcagctctataaaaatggggacagcccctgcttcaatgacaattttggtctgctgagaggttccagaggcaatattcgttagagcccaggcagcttcaaactgtaatgtacaattctcattcctcttcagaaactccacgaaccgatccaccactcttggagtgttgataacttcatctattggaggactaggctctttggagagcagtttccggaatttctgtgtggttgctaactgcaggtcagaatcatcagaaaagagcatctccaccatctctcttgtgatcacactctccccagtggtagagctcacataagagtccatgagaagactatcgaacatggcagcttcttcattaatcagctccacatttctccgtttaaaaagttgttgctctcgcttctgcttccggagctgaatgccctcttcctctcttcttcgtctcatttcttcagggtttagagcattgttcttatagctcttcattcgataattgtctttccctgggctcgccatggtctctgacacatagcttttcatgactgagcctgggctgtcctggacgctagcctctccttcaagcacagctgacagtgaagctgggaggagagccatgctgagcttctttagtcaccatggtgacaagaaactatcacaaatatttgcttatgacttcactggggaagcagacaagggaggttagattggaaggaggaacatctgcacaagcacatctggaatctcagggatccagcacgccagcggctttttccattatgtactcccttacttgctgtggatgaattttttaaaattcacaatacaaataaacttttctagcatctggctgtcctagactgtctttgggttttcttagtcaaggaactctctcaaagtgaataggtctctgaagtcacacctttcatttctagggaatgtctaatgttgccatgcactttctaagcttttaaaac

SEQ ID NO: 14248 - RNA, 6708 nt, Homo sapiens
  source 1..6708: mol_type = other RNA
gctgggattacaggcatgagccaccgcgcccagctgaagatgtggattttttttttttttttttttttgagatggagtctcgcactgtcacccaagctggagtgcagtggcatgatcttggctcactgcaacctccgcctcctgggttcaagtgattctcctgtctcagcctcccaagtagctgggattacaggcgcctgccaccacgcccagctaattttttgtatttttattagagatggggtttcactatgttgccaggctggtctcaaactcctgacctcgtgatccacccgcctcggcctcccaaagtgctgggattacaggcatgtgccaccgcgcctggccagatgtggactctttaaagacatgctctgagtcagaggttcccagccagtgttaggatctctgagagcttacttccttcaatgccccccaggccatggcgtatataatagttacaggagaacagggctggcattcagcaacagggttcaggtacgagctaatgtggacatcagaagtcagcctggcccagaggcagctaggcaggccactaagatacactacataaaccttttcccatggtgttctgggcctaacatgtaatactgcctcttctaactctcacagcctgcttaggttctgcacatagcccagacctgaagcaaagcgcccttgcagagaaaaaaataacagctttaattcacagatttggttggtcttgacctcaagttcttcctttgccacggtctaaatcagggtgtggggctagaggacagataatgagagactgaatcatttatgaaggccttggccaaagagcagctagtgcccactacatggatcccagcagggccaaattctcaacttgttggcttaacaaaagaatgaaaaagctcaaacagaaaacatactggacaaggttggtccagaacatgcaatcctaaatggctatggaataaatttattctgagcaatatctcagtctcacactcactaaattctagggtagttctattgaagatgtttaccatggtttagcgcactgagccctgcacccttccccaggctgccagggaagcagagaggtacaaacattcctaatgccccagtcagcctgttctccctatggggtccctggattacctgcagggacctgggggaaattggctccctgtcttcagctgagagtctggaatctgaaccctagatgaatctactgaagaatgctcaagatgatggataccaagctgagtgagtctaggggagaagagaggcctgaacaaaagagctggggccttcaaagaggtgtatgagaggtgaggttagtagtgccaggctttcctatcttttccttctagtttgctagaaacaagtacaactttagggtgtggggggaaggcaggtagacatgaagaaatggaaatacagttcattctgctagacattttaaactggtttggcttgagaaaaatagaaagtctgtgcctgagaaccttcttttcctctcccttatttaagtacaatagcagctataatctgtgcagttcagctccaaaaaacagggctcctggaagatggctttcatggcagagagttgatggggtagattaatgggctctaggtaaggagcaacaccaagggtccctgaaaactgaggccaacacctgctccctgggggggggccatttgtattccctgacccatgtaacaagcctggccagctgtgggtggaatccatgtggttctatcagaaggctgcagccaacatcaaggccaggcagtcaccagggtcagctgggatctgaagggaggcttctaagaccagacaccctgttagtactaaagatgatgatttgggggtgggatgcctggaggggctggcaccattcaaaaaagtattggaaaacattagccaagaaaaaggctccttgtccctcctaatccatatccagatacccccaaccagagatcttaaaaaggatagaccagccatatgccaacatgccaggattccaaaagcatgcctcaactaattagggtattccctacagcagactggggtagaggggctccatcctggcaataaccagagagccttacctcgcctaggccagggtatggaatctagatgaagactgtccacaaacagtggctctcaagcctgggctaaataaataatattttgcttcattacatggccaaaggagaggaggagatagaaaagatgatattactacctctgtgggctggaagaacttcacctgttggttgaaaggggattaaaggaagataacaggaaaacctggtctggagaagacataaatgaaagctcctggaggccacttttctctgattagaaatctatcctcacactctgcccctagtagactttagcctttggagttcttagggaaaactggctttaagcagcagccagatcaccaaaaacattttccatctggtacaggacccggagctgaagccaaagtagattttggaggaacagctggacaagcaggatgtgtatgtcttacactaagaaactggtccctgtatcagggacttaactcttacttgagatgtacaaagtagatcctactaaattgccctttggaagagaacaatgggcggaggttgggtaggggaaggctttttttttttttttttttttaaactgtaagagaatggttttttaatggaggtagcaggccaagtgaaaaaaagattctgccccctgccttcctgggagattgggagttggcagccatcattcccaagctgatgagtggcatatgactcaccaaggtggtacaacatgggtgggatttttcaaggacaattgccagacctaaaccatcctcctcagaaaatggctttgaagtgggactgcagcactaggagagggcaaattcaagatcaatggccaataataagtacctgaactttaggtctataagcagaagggcatggatttcacctgagccagaaggagatgtgtagcaatagaagcaagaatggcattgtttcagaggaaggaaaagcagagcttggagcaggatgcctctgactaaccacagtggggaggtgggggtggggcagactgtgccttcagctccacagctggtctacaccaacttcctctactcccatccaaacaggtgggctttactatcatatgtaatccacccagaggcacaggcaagccactaaggcaatgcactaccgtaattcaaacagaaagaagaggcatctggattataattgtcacaaggaagggaaaacccaaaccaggtacaaggatcccaaacagggaagatacgcaatagctctaaaaaaaaaaaaaaaaaaagcaggctactaagtttcagtgataatagataataggagaggcagccatgggtgatcagttatgtggacaatggccattgagattgaatttgacaaggcaaactgcttctgagtttcctgatacaagcaggatgttcagcagtaaggacagagtagcagacttcaccaggccctgaggccatccttgctcccttcaggtcctgggacaatcaggccacgctgacctgctttatgaaggttccagagctgaaggttggtcccaggtggtggtccagaatccaagcagagaggaaaaggaccaagctcaggcctcctgagcgaggaagcatccatatctctttttggtcttcctcacagtatcctacttaccgaaatgacagacagttcttcctcttgagaccaattaagattgacctacctaatatatagaatataaaaaaatacagaactttttgacattctctcctttagaagtaaaatatacatgatccaactatggaagaggaagaagaagaagaagaaaggccaaaggcagggatccctgactatcccaatacatgacactctcactccaccctcctctgcaacttacaggtcaccagagcaaggactttctcctcaggagaaaggaaggaccacagccccctatctcaagcttaggagaaaatacagccacctcagaggttctctcaacctcgagggggaattttcaagtaaacaaatgaagttgggtcgcaccatttggaaggtgagtaggaaatatgggatcagtagctacacgtgggaagccccatctgaaggcctgtgctcctcccctgcactcccactggtatacttgagacacttcaggagagtgaggaggatcccccaaactaaagaggtctgggcaaagagtcagagggagggagggacctttgtttcatggtagcctccccagcctctagtcccaggcaatgcaggcagctgggtttactaaaaccaggaacttgtggctcttgggaagagcaatcttaatacaagaaaaatgtgcaaaagaaaaaaaaattaaataactcaatccaagcgtacaagattaatattctgtcagagcaagaacactttgttttggatttctcccttcccctcccacctcccacctctggaatataccgtctgctcaagtacccaagataagagttacacagatcagggcagaggaccgggaagaatgaaaaaagataaagggaaggaagtcaccactgaagaaaaaaagaaaaaaaataaaaataaaaaaaggtgcaaattgattaccttagtcctcctttgtctacccctgggctcctgggttaaagacatgtgtgcagccaaaatatagtgtaaggaagaaaaacccaacacgtccccttcttgtcacaaaacccaaaggtgagcctcagatggttctgtctgtccagagggtgctccctccagggaagggggcggagcaggtcaagagcacagtctccagggcagcagaggtgtgtggtggctgatggtggggacactggtttcccgcccaccagagggctgctcttccgctggctggtggtgcttcccatcccctcccctccctggaggcagatattatagctggaagccctccatgggggcctcaggctgctggaagatgaactgctgttgcgtttcatcgacttggggagccaggctgctatcatcgtcttctacaccaaagtagtgctcaatgaggtcgaaggccttctggtagatctcctggttctcgtggctctggagaaactcaattttatccaagccataggcttcctctatgaggccacaataaggattgacccctgagccactgcgcttgccctcttgctctccaagccgcaggatgttctccagtccattgagggccacttgcacaatcttcgaatccattacagtcagcaagtcacataggggtttgatgcagcccagtgagaccaggtacctgatctgctcaggggttcctcctgatgtggcattggtgatggcccaggctgcctctttccttgtacgaaactctgctttctgaaggatttcgatcaacacagggaagatatttgcatctataacagcctgtatttgagccctgttgccagcagtaatatttgaaatagtccagcaagcttccttccggattgactccttgggactgctcaacaagtggagaaggcaaggtagggctgaacagttaagaatgacctgggtctggatgtcatccccagtgacgatgttacccacggctctcagggcaggagaagccactttgtaatcattgtgcatcagcagctctaccaatctccggcagactccggagtctatgactgcctggatcttctcattggggccatcagacagataagaaagggcccagcaagcatctgccagcaagtccgagtcgctgctgaagagtaggcgagacagtacaggcaaacaaggagagacctttgcaaactctgggggtgggtttttccctcggcagagatttgacagggcccagactgcattccgtgtcatcgtcagtcgtgtggacttggtaaggagtgttaacaaaggattaaggatggaacagttcaagacgtaatctcggcaaacagagctatctccagctatgtttcccagtgcccagactgcctgttcctgaacatcctcaaagtctgaattaagcagctctataaaaatggggacagcccctgcttcaatgacaattttggtctgctgagaggttccagaggcaatattcgttagagcccaggcagcttcaaactgtaatgtacaattctcattcctcttcagaaactccacgaaccgatccaccactcttggagtgttgataacttcatctattggaggactaggctctttggagagcagtttccggaatttctgtgtggttgctaactgcaggtcagaatcatcagaaaagagcatctccaccatctctcttgtgatcacactctccccagtggtagagctcacataagagtccatgagaagactatcgaacatggcagcttcttcattaatcagctccacatttctccgtttaaaaagttgttgctctcgcttctgcttccggagctgaatgccctcttcctctcttcttcgtctcatttcttcagggtttagagcattgttcttatagctcttcattcgataattgtctttccctgggctcgccatggtctctggaattctgaaatcaaaggggctctcagggccaggcacgatggctcatacctataattctagcactttaggaggccgaggcaggaggattgcttgaggccaggagtttgcaaccagcctaggcaactaagcaagacccaatct

SEQ ID NO: 14249 - RNA, 4889 nt, Homo sapiens
  source 1..4889: mol_type = other RNA
gctgggattacaggcatgagccaccgcgcccagctgatttatatcttatctatgagaaacaccaaaaactatgagtaagcatcactgagttatcatgtaagaattttttctaagttttagcccaaatttccaggtcaagacaaacccacagagaggtaaaagggtattaggatgggagttcatatttacagcaggaactttacatacatggtctccttgagctcttgcaaccttgtaagataagtattattttcctttcacagatgaataaactgctaccctttttttaacaagtagatttgactaaaaagaactatgtcaaatattgcttcccattttcttatttcttttttttttttttttgagacagagtcttgctctgttgcccaggctggagtgcagtggcgagatctcggctcactgcaagctctgcctcccgggttcacaccattctcctgcctcagcctcccgagtagctgggactacaggcgcccgccaccacgcccggctaattttctgttttttagtagagacggggtttcaccgtgttagccaggatggtctcgatctcctgacctcgtgatccacctgcctcagcctcccaaagtgctgggattacaggcgtgagccactgagcccagccccattttatttcatttctctaacagcaatgatatatatacatcccatagtatatcctactgatatactagcccctttccccattcaacacctgtgtaatcaggaaataaaacaatgattcgggtttaaagggtatatcatgtgaaactaatgctggggcggtagtctccattcatagttcaaaatacaaattttatccactaaaatggaaacacaaaaaacaactactgaaatgtaaataatataacaacaaaaataacaaaatatcataatacacagggccaaatcacattatatacactcactacacccactctaccctaccttagcccgtaatcaaagggacaggggaaaaaaccaaatgtagcaggaaaggcaatataaagctattaattaattaactggaatttagtttgtaaatgctaaaaccagttctcaaaaattaagacaatgcttttgatcagcagactaaattattacaaataaagataagtacttattgcaaaactacttgaatctttgcatgactaaaatgtaaaataagtggtgacttgaaatcctagagtgaactttatacagaaaaggaatagtctacatgtagacactgagaactcttgggagggggaaaagatttggatatggctatagttttgactttgcaaatgatcaatttttgcggaattagatggaaaagatccggtgctttttatagttcaaacacagacaaatgctgttaagtctccaaaaatttgattagaagttggagtgctgagtgattttaagaacctgaagcaacagcatttctaaacaattcttaaaataaacttgttagccacatcagcgttgtgcattaaatttcacaactcatggagaggaagaaaaaaagtcttgcttaactctaaacatacaagttttagaagaattttaatgaagtgcggctcccagaacaggaaaagccttatgttaaaacaattcagtccttgagtccttggctaacaactagattgaactacctacctgacttggaagtgaagtgtcctggaaaacatattttaaaaattttaacacttttctccccttgtagaaaactttaaatttaaagtctagactatacagaccaaattcaagttaatgactatataaccaaactaagtggcagacagtgcaaaggtgaagaactgaggatttacatactaaaacagaaacagggcagtcattatttaatttttaaaactctcatttaaatttgcaatgttttagccgggcgtggtggctcaagcctgtaatcccagcactttgggagggcaaggcgagtggatctcttgaggtcaggagtttgataccagcctggccaacatggtgaaaccccgtctctactaaaaataaaaaaaaattagtcgggcatggtggcacctgcctgtaattccagctactcaggaagctgaggcacgagaatcgcttgaacccagaaggcggaggttgcagtgagcagagatcactccactgcactccagcctgggtgacaagcaagactccatctcaaaaagaaaattaaataaataaaataaatttgcaatgttttaaatgaatatcacttaaagtagtaatcaacagaagttaggagaacataacaatactctttctcttagaaagtacaacaaaaatataattttttacagttttactctcaaactttcctctgtagtaacatgccttactcacctctacaataggtttgttgtgagaatcttgtaatgtaaaccctggacgttctatgaagcatttttaaacttctagtttataccctactgattcttattcaagtgttttttaaaaaatatttaaacaactattcttcttttcttgccaatatttttataatttccaagaggttttaaggatcttgagagaacatttatttcagaagtatctactactattactagccaagaaaacaaatgtaggtagaggaaagacttaacattttgtcctatatacatcttaatcatcctaacggtaaaaactcacatgaaactttaagatacaagatgatatgagaatctcaacatggaaagctgtcactataactacaagcagtgtacaaacatgcttctacttttacctacataagctgacagatgtttaaaatactgagttaacaaagatcttttagtaaagtgacttaggcaggcttaaactagcaaggattaaggatgaatccttactaattaattggaagatctgagacatattttatatttcattttacaaaatcagaaatacttattttgaaacaagataagacatggtctacctgtcaaaaaactaccactcagaaatatttttcatccacaaagcaggaaaaacataaaatcatttacatttcacattggcaccaaaaaggttaactgccctgccttcttggattagaaaaactaaagctgagtgataagtagttttgcaggcgtttgaacatgcctaagcctttaaatcagcaaaatactttctaaaaattctgattacaaaagtaatacatacttataaaaaattcgaacagaacaaaatgaaaaaagtagaaagtgaaaaggcccctataaaacccctctggggcccctcccccaatccccccctccccgaagagaaaccacatttaacagtttggtgtatatctttccaaatcttttgttctatgcatattaaaaacatacatactttgatctggctcagactatacatagtgttttgccacttgcattttacacttaacatatctttgacatctttccatgtcagtacatgttggctcgatagtattctatcattaaatacgctttcaaaaatggcaaatcactttaaaaaaataattcgcacaagtacgtgtttataactttaaaagaaaatggacagaatcctaaaacacaacaaccaacctctaaaaacaatctctatctttccaccagcatggaacaatttattcctttttcacacaaaacaaattatgtgattggggagattaactctaatctccacatttatatacagaaagctccatttgttaagcctatctgaaaagaataaaaaatccagatgattaattcacttacacttagaaattaaatcagtatactatgaatacacattgtgttcagttatagtatgatgcttcttattcttagtctatggtttcaattaaataacagtaaaaaaaatggataatacagctaataccctgaaaaatcaagaaattcaaagattatattgccaactaaaacactgccatgtacattttttttcctacttggtagcaaatgctaatggaattcaatcctgattacttaaagtcagttcacatcacacattcaatcagggtaataagaacaacataacatgcctactatagagttagattaagacataaaaattttttgcttgaaagtaatgactgtgtagcacatgggacacttgtcaactgcttcagcacattgtttacaagtgactagatgtccacaaggaacaaaaacgatagcaatatttctatccatacagattttgcaaagcttctcctcttgcaggcgccttagctgctcttcagtactaatctctttctgtaatgaagtctgacttgactcatcttgcatactgtctttctgagcattcactagatctgcaaccagaacctcaagtgatttatagttgctcccagatatctgaattttttcctccattattttcttaatgtccttgaaactgaaccccattcgtatagcttcttgtaccataggattttggaagatggtatcatcaattcttctagttagtgatggtgttttctcagtagttcttaccagacactcctcaagtgaatgagttaaatgaatattgtttatatattcttgtcccttctgttctaacagatatttgcaccctggataccatttagcatgttgttcccaagggtcttcactgggcttccaatcagttagccctcctccacagtgaaagcactttactttatcaccttcaccgcgccaggacagccggcccgaactgccccgcggcgatcggctcggtccaaggggagggtcccggaggaggcgcggcccgagccccaatctggaaatgccaactccgctctgcggcttggccccagccacttgggccgggcgtccctcgatgagcgccacgccggctccgggcgccgccaaggtcccgccacctagcgcgcgcacatgcgcagtgagcacctc

SEQ ID NO: 14250 - RNA, 4907 nt, Homo sapiens
  source 1..4907: mol_type = other RNA
gctgggattacaggcatgagccaccgcgcccagctgatttatatcttatctatgagaaacaccaaaaactatgagtaagcatcactgagttatcatgtaagaattttttctaagttttagcccaaatttccaggtcaagacaaacccacagagaggtaaaagggtattaggatgggagttcatatttacagcaggaactttacatacatggtctccttgagctcttgcaaccttgtaagataagtattattttcctttcacagatgaataaactgctaccctttttttaacaagtagatttgactaaaaagaactatgtcaaatattgcttcccattttcttatttcttttttttttttttttgagacagagtcttgctctgttgcccaggctggagtgcagtggcgagatctcggctcactgcaagctctgcctcccgggttcacaccattctcctgcctcagcctcccgagtagctgggactacaggcgcccgccaccacgcccggctaattttctgttttttagtagagacggggtttcaccgtgttagccaggatggtctcgatctcctgacctcgtgatccacctgcctcagcctcccaaagtgctgggattacaggcgtgagccactgagcccagccccattttatttcatttctctaacagcaatgatatatatacatcccatagtatatcctactgatatactagcccctttccccattcaacacctgtgtaatcaggaaataaaacaatgattcgggtttaaagggtatatcatgtgaaactaatgctggggcggtagtctccattcatagttcaaaatacaaattttatccactaaaatggaaacacaaaaaacaactactgaaatgtaaataatataacaacaaaaataacaaaatatcataatacacagggccaaatcacattatatacactcactacacccactctaccctaccttagcccgtaatcaaagggacaggggaaaaaaccaaatgtagcaggaaaggcaatataaagctattaattaattaactggaatttagtttgtaaatgctaaaaccagttctcaaaaattaagacaatgcttttgatcagcagactaaattattacaaataaagataagtacttattgcaaaactacttgaatctttgcatgactaaaatgtaaaataagtggtgacttgaaatcctagagtgaactttatacagaaaaggaatagtctacatgtagacactgagaactcttgggagggggaaaagatttggatatggctatagttttgactttgcaaatgatcaatttttgcggaattagatggaaaagatccggtgctttttatagttcaaacacagacaaatgctgttaagtctccaaaaatttgattagaagttggagtgctgagtgattttaagaacctgaagcaacagcatttctaaacaattcttaaaataaacttgttagccacatcagcgttgtgcattaaatttcacaactcatggagaggaagaaaaaaagtcttgcttaactctaaacatacaagttttagaagaattttaatgaagtgcggctcccagaacaggaaaagccttatgttaaaacaattcagtccttgagtccttggctaacaactagattgaactacctacctgacttggaagtgaagtgtcctggaaaacatattttaaaaattttaacacttttctccccttgtagaaaactttaaatttaaagtctagactatacagaccaaattcaagttaatgactatataaccaaactaagtggcagacagtgcaaaggtgaagaactgaggatttacatactaaaacagaaacagggcagtcattatttaatttttaaaactctcatttaaatttgcaatgttttagccgggcgtggtggctcaagcctgtaatcccagcactttgggagggcaaggcgagtggatctcttgaggtcaggagtttgataccagcctggccaacatggtgaaaccccgtctctactaaaaataaaaaaaaattagtcgggcatggtggcacctgcctgtaattccagctactcaggaagctgaggcacgagaatcgcttgaacccagaaggcggaggttgcagtgagcagagatcactccactgcactccagcctgggtgacaagcaagactccatctcaaaaagaaaattaaataaataaaataaatttgcaatgttttaaatgaatatcacttaaagtagtaatcaacagaagttaggagaacataacaatactctttctcttagaaagtacaacaaaaatataattttttacagttttactctcaaactttcctctgtagtaacatgccttactcacctctacaataggtttgttgtgagaatcttgtaatgtaaaccctggacgttctatgaagcatttttaaacttctagtttataccctactgattcttattcaagtgttttttaaaaaatatttaaacaactattcttcttttcttgccaatatttttataatttccaagaggttttaaggatcttgagagaacatttatttcagaagtatctactactattactagccaagaaaacaaatgtaggtagaggaaagacttaacattttgtcctatatacatcttaatcatcctaacggtaaaaactcacatgaaactttaagatacaagatgatatgagaatctcaacatggaaagctgtcactataactacaagcagtgtacaaacatgcttctacttttacctacataagctgacagatgtttaaaatactgagttaacaaagatcttttagtaaagtgacttaggcaggcttaaactagcaaggattaaggatgaatccttactaattaattggaagatctgagacatattttatatttcattttacaaaatcagaaatacttattttgaaacaagataagacatggtctacctgtcaaaaaactaccactcagaaatatttttcatccacaaagcaggaaaaacataaaatcatttacatttcacattggcaccaaaaaggttaactgccctgccttcttggattagaaaaactaaagctgagtgataagtagttttgcaggcgtttgaacatgcctaagcctttaaatcagcaaaatactttctaaaaattctgattacaaaagtaatacatacttataaaaaattcgaacagaacaaaatgaaaaaagtagaaagtgaaaaggcccctataaaacccctctggggcccctcccccaatccccccctccccgaagagaaaccacatttaacagtttggtgtatatctttccaaatcttttgttctatgcatattaaaaacatacatactttgatctggctcagactatacatagtgttttgccacttgcattttacacttaacatatctttgacatctttccatgtcagtacatgttggctcgatagtattctatcattaaatacgctttcaaaaatggcaaatcactttaaaaaaataattcgcacaagtacgtgtttataactttaaaagaaaatggacagaatcctaaaacacaacaaccaacctctaaaaacaatctctatctttccaccagcatggaacaatttattcctttttcacacaaaacaaattatgtgattggggagattaactctaatctccacatttatatacagaaagctccatttgttaagcctatctgaaaagaataaaaaatccagatgattaattcacttacacttagaaattaaatcagtatactatgaatacacattgtgttcagttatagtatgatgcttcttattcttagtctatggtttcaattaaataacagtaaaaaaaatggataatacagctaataccctgaaaaatcaagaaattcaaagattatattgccaactaaaacactgccatgtacattttttttcctacttggtagcaaatgctaatggaattcaatcctgattacttaaagtcagttcacatcacacattcaatcagggtaataagaacaacataacatgcctactatagagttagattaagacataaaaattttttgcttgaaagtaatgactgtgtagcacatgggacacttgtcaactgcttcagcacattgtttacaagtgactagatgtccacaaggaacaaaaacgatagcaatatttctatccatacagattttgcaaagcttctcctcttgcaggcgccttagctgctcttcagtactaatctctttctgtaatgaagtctgacttgactcatcttgcatactgtctttctgagcattcactagatctgcaaccagaacctcaagtgatttatagttgctcccagatatctgaattttttcctccattattttcttaatgtccttgaaactgaaccccattcgtatagcttcttgtaccataggattttggaagatggtatcatcaattcttctagttagtgatggtgttttctcagtagttcttaccagacactcctcaagtgaatgagttaaatgaatattgtttatatattcttgtcccttctgttctaacagatatttgcaccctggataccatttagcatgttgttcccaagggtcttcactgggcttccaatcagttagccctcctccacagtgaaagcactttactttatcaccttcaccgcgccaggacagccggcccgaactgccccgcggcgatcggctcggtccaaggggagggtcccggaggaggcgcggcccgagccccaatctggaaatgccaactccgctctgcggcttggccccagcctaggtgaaggaaacggaagtcccttcgtctccctcacgcgcctctaccggccggcccatcccctggagaaacccggagtcgtgaaacccgaagtgtgtccacgtcagggcctc

SEQ ID NO: 14251 - RNA, 5667 nt, Homo sapiens
  source 1..5667: mol_type = other RNA
gctgggattacaggcatgagccaccgcgcccagctgatttatatcttatctatgagaaacaccaaaaactatgagtaagcatcactgagttatcatgtaagaattttttctaagttttagcccaaatttccaggtcaagacaaacccacagagaggtaaaagggtattaggatgggagttcatatttacagcaggaactttacatacatggtctccttgagctcttgcaaccttgtaagataagtattattttcctttcacagatgaataaactgctaccctttttttaacaagtagatttgactaaaaagaactatgtcaaatattgcttcccattttcttatttcttttttttttttttttgagacagagtcttgctctgttgcccaggctggagtgcagtggcgagatctcggctcactgcaagctctgcctcccgggttcacaccattctcctgcctcagcctcccgagtagctgggactacaggcgcccgccaccacgcccggctaattttctgttttttagtagagacggggtttcaccgtgttagccaggatggtctcgatctcctgacctcgtgatccacctgcctcagcctcccaaagtgctgggattacaggcgtgagccactgagcccagccccattttatttcatttctctaacagcaatgatatatatacatcccatagtatatcctactgatatactagcccctttccccattcaacacctgtgtaatcaggaaataaaacaatgattcgggtttaaagggtatatcatgtgaaactaatgctggggcggtagtctccattcatagttcaaaatacaaattttatccactaaaatggaaacacaaaaaacaactactgaaatgtaaataatataacaacaaaaataacaaaatatcataatacacagggccaaatcacattatatacactcactacacccactctaccctaccttagcccgtaatcaaagggacaggggaaaaaaccaaatgtagcaggaaaggcaatataaagctattaattaattaactggaatttagtttgtaaatgctaaaaccagttctcaaaaattaagacaatgcttttgatcagcagactaaattattacaaataaagataagtacttattgcaaaactacttgaatctttgcatgactaaaatgtaaaataagtggtgacttgaaatcctagagtgaactttatacagaaaaggaatagtctacatgtagacactgagaactcttgggagggggaaaagatttggatatggctatagttttgactttgcaaatgatcaatttttgcggaattagatggaaaagatccggtgctttttatagttcaaacacagacaaatgctgttaagtctccaaaaatttgattagaagttggagtgctgagtgattttaagaacctgaagcaacagcatttctaaacaattcttaaaataaacttgttagccacatcagcgttgtgcattaaatttcacaactcatggagaggaagaaaaaaagtcttgcttaactctaaacatacaagttttagaagaattttaatgaagtgcggctcccagaacaggaaaagccttatgttaaaacaattcagtccttgagtccttggctaacaactagattgaactacctacctgacttggaagtgaagtgtcctggaaaacatattttaaaaattttaacacttttctccccttgtagaaaactttaaatttaaagtctagactatacagaccaaattcaagttaatgactatataaccaaactaagtggcagacagtgcaaaggtgaagaactgaggatttacatactaaaacagaaacagggcagtcattatttaatttttaaaactctcatttaaatttgcaatgttttagccgggcgtggtggctcaagcctgtaatcccagcactttgggagggcaaggcgagtggatctcttgaggtcaggagtttgataccagcctggccaacatggtgaaaccccgtctctactaaaaataaaaaaaaattagtcgggcatggtggcacctgcctgtaattccagctactcaggaagctgaggcacgagaatcgcttgaacccagaaggcggaggttgcagtgagcagagatcactccactgcactccagcctgggtgacaagcaagactccatctcaaaaagaaaattaaataaataaaataaatttgcaatgttttaaatgaatatcacttaaagtagtaatcaacagaagttaggagaacataacaatactctttctcttagaaagtacaacaaaaatataattttttacagttttactctcaaactttcctctgtagtaacatgccttactcacctctacaataggtttgttgtgagaatcttgtaatgtaaaccctggacgttctatgaagcatttttaaacttctagtttataccctactgattcttattcaagtgttttttaaaaaatatttaaacaactattcttcttttcttgccaatatttttataatttccaagaggttttaaggatcttgagagaacatttatttcagaagtatctactactattactagccaagaaaacaaatgtaggtagaggaaagacttaacattttgtcctatatacatcttaatcatcctaacggtaaaaactcacatgaaactttaagatacaagatgatatgagaatctcaacatggaaagctgtcactataactacaagcagtgtacaaacatgcttctacttttacctacataagctgacagatgtttaaaatactgagttaacaaagatcttttagtaaagtgacttaggcaggcttaaactagcaaggattaaggatgaatccttactaattaattggaagatctgagacatattttatatttcattttacaaaatcagaaatacttattttgaaacaagataagacatggtctacctgtcaaaaaactaccactcagaaatatttttcatccacaaagcaggaaaaacataaaatcatttacatttcacattggcaccaaaaaggttaactgccctgccttcttggattagaaaaactaaagctgagtgataagtagttttgcaggcgtttgaacatgcctaagcctttaaatcagcaaaatactttctaaaaattctgattacaaaagtaatacatacttataaaaaattcgaacagaacaaaatgaaaaaagtagaaagtgaaaaggcccctataaaacccctctggggcccctcccccaatccccccctccccgaagagaaaccacatttaacagtttggtgtatatctttccaaatcttttgttctatgcatattaaaaacatacatactttgatctggctcagactatacatagtgttttgccacttgcattttacacttaacatatctttgacatctttccatgtcagtacatgttggctcgatagtattctatcattaaatacgctttcaaaaatggcaaatcactttaaaaaaataattcgcacaagtacgtgtttataactttaaaagaaaatggacagaatcctaaaacacaacaaccaacctctaaaaacaatctctatctttccaccagcatggaacaatttattcctttttcacacaaaacaaattatgtgattggggagattaactctaatctccacatttatatacagaaagctccatttgttaagcctatctgaaaagaataaaaaatccagatgattaattcacttacacttagaaattaaatcagtatactatgaatacacattgtgttcagttatagtatgatgcttcttattcttagtctatggtttcaattaaataacagtaaaaaaaatggataatacagctaataccctgaaaaatcaagaaattcaaagattatattgccaactaaaacactgccatgtacattttttttcctacttggtagcaaatgctaatggaattcaatcctgattacttaaagtcagttcacatcacacattcaatcagggtaataagaacaacataacatgcctactatagagttagattaagacataaaaattttttgcttgaaagtaatgactgtgtagcacatgggacacttgtcaactgcttcagcacattgtttacaagtgactagatgtccacaaggaacaaaaacgatagcaatatttctatccatacagattttgcaaagcttctcctcttgcaggcgccttagctgctcttcagtactaatctctttctgtaatgaagtctgacttgactcatcttgcatactgtctttctgagcattcactagatctgcaaccagaacctcaagtgatttatagttgctcccagatatctgaattttttcctccattattttcttaatgtccttgaaactgaaccccattcgtatagcttcttgtaccataggattttggaagatggtatcatcaattcttctagttagtgatggtgttttctcagtagttcttaccagacactcctcaagtgaatgagttaaatgaatattgtttatatattcttgtcccttctgttctaacagatatttgcaccctggataccatttagcatgttgttcccaagggtcttcactgggcttccaatcagttagccctcctccacagtgaaagcactttactttatcaccttcacctaaagcataaaatccagctcttgcaagctgctccttgttaactgagtatatccatgtcccaaaagtaaagatccgtgcttcataatctgccatggatggatttcttggaagatttgttgaatttgggaaattcctatcagaactcacagcatcagattcacttcgaatattaagattccggcccaaaacaaagaagcaattaggaaagtgtcgcctgtgttctgaccaggcacgatcacaaggttcccaatttttcagttttccaccacaacaaaagcactgcacttggtcaccaatacctgtgtagtagagtccagcacttgctaactctcttggggttaggtgagcatagtctggccagttctgaaaggactttaatctagcttcttcactatacatggcagggttcctcgggtatatggtgtctgatatatctacaacctgcccagttctcaaaagatagtctgcatgtgtctcagatggcctgtctaaggcaaaatgatctctgcttcccagatagttttcaactttgtactgaccattctggataccagaatttgtagactgcgtggcactattttcaagataaaagccgttgataaatctgcaatttggggatactttcctgtgtcttccaactgctgagtctccatattgccatctatctacagctgcatgacaactaaagcaccgcacggtatctccttcaccagtataaagaaaccctgctcgtgccagtgttgatgctgaaacaggactaccacttggaaaattagcaaaagtttttaatctattaaactcttctacaaattcttcttccttattgatgtctgcaggtacacaagttttagatccttcaaaactgttaaaagtcatcttctcttgaaaataggacttgtccaccttttcacttgggccgggcgtccctcgatgagcgccacgccggctccgggcgccgccaaggtcccgccacctccccgaaccggatgggggcagtaag

SEQ ID NO: 14252 - RNA, 5794 nt, Homo sapiens
  source 1..5794: mol_type = other RNA
gctgggattacaggcatgagccaccgcgcccagctgatttatatcttatctatgagaaacaccaaaaactatgagtaagcatcactgagttatcatgtaagaattttttctaagttttagcccaaatttccaggtcaagacaaacccacagagaggtaaaagggtattaggatgggagttcatatttacagcaggaactttacatacatggtctccttgagctcttgcaaccttgtaagataagtattattttcctttcacagatgaataaactgctaccctttttttaacaagtagatttgactaaaaagaactatgtcaaatattgcttcccattttcttatttcttttttttttttttttgagacagagtcttgctctgttgcccaggctggagtgcagtggcgagatctcggctcactgcaagctctgcctcccgggttcacaccattctcctgcctcagcctcccgagtagctgggactacaggcgcccgccaccacgcccggctaattttctgttttttagtagagacggggtttcaccgtgttagccaggatggtctcgatctcctgacctcgtgatccacctgcctcagcctcccaaagtgctgggattacaggcgtgagccactgagcccagccccattttatttcatttctctaacagcaatgatatatatacatcccatagtatatcctactgatatactagcccctttccccattcaacacctgtgtaatcaggaaataaaacaatgattcgggtttaaagggtatatcatgtgaaactaatgctggggcggtagtctccattcatagttcaaaatacaaattttatccactaaaatggaaacacaaaaaacaactactgaaatgtaaataatataacaacaaaaataacaaaatatcataatacacagggccaaatcacattatatacactcactacacccactctaccctaccttagcccgtaatcaaagggacaggggaaaaaaccaaatgtagcaggaaaggcaatataaagctattaattaattaactggaatttagtttgtaaatgctaaaaccagttctcaaaaattaagacaatgcttttgatcagcagactaaattattacaaataaagataagtacttattgcaaaactacttgaatctttgcatgactaaaatgtaaaataagtggtgacttgaaatcctagagtgaactttatacagaaaaggaatagtctacatgtagacactgagaactcttgggagggggaaaagatttggatatggctatagttttgactttgcaaatgatcaatttttgcggaattagatggaaaagatccggtgctttttatagttcaaacacagacaaatgctgttaagtctccaaaaatttgattagaagttggagtgctgagtgattttaagaacctgaagcaacagcatttctaaacaattcttaaaataaacttgttagccacatcagcgttgtgcattaaatttcacaactcatggagaggaagaaaaaaagtcttgcttaactctaaacatacaagttttagaagaattttaatgaagtgcggctcccagaacaggaaaagccttatgttaaaacaattcagtccttgagtccttggctaacaactagattgaactacctacctgacttggaagtgaagtgtcctggaaaacatattttaaaaattttaacacttttctccccttgtagaaaactttaaatttaaagtctagactatacagaccaaattcaagttaatgactatataaccaaactaagtggcagacagtgcaaaggtgaagaactgaggatttacatactaaaacagaaacagggcagtcattatttaatttttaaaactctcatttaaatttgcaatgttttagccgggcgtggtggctcaagcctgtaatcccagcactttgggagggcaaggcgagtggatctcttgaggtcaggagtttgataccagcctggccaacatggtgaaaccccgtctctactaaaaataaaaaaaaattagtcgggcatggtggcacctgcctgtaattccagctactcaggaagctgaggcacgagaatcgcttgaacccagaaggcggaggttgcagtgagcagagatcactccactgcactccagcctgggtgacaagcaagactccatctcaaaaagaaaattaaataaataaaataaatttgcaatgttttaaatgaatatcacttaaagtagtaatcaacagaagttaggagaacataacaatactctttctcttagaaagtacaacaaaaatataattttttacagttttactctcaaactttcctctgtagtaacatgccttactcacctctacaataggtttgttgtgagaatcttgtaatgtaaaccctggacgttctatgaagcatttttaaacttctagtttataccctactgattcttattcaagtgttttttaaaaaatatttaaacaactattcttcttttcttgccaatatttttataatttccaagaggttttaaggatcttgagagaacatttatttcagaagtatctactactattactagccaagaaaacaaatgtaggtagaggaaagacttaacattttgtcctatatacatcttaatcatcctaacggtaaaaactcacatgaaactttaagatacaagatgatatgagaatctcaacatggaaagctgtcactataactacaagcagtgtacaaacatgcttctacttttacctacataagctgacagatgtttaaaatactgagttaacaaagatcttttagtaaagtgacttaggcaggcttaaactagcaaggattaaggatgaatccttactaattaattggaagatctgagacatattttatatttcattttacaaaatcagaaatacttattttgaaacaagataagacatggtctacctgtcaaaaaactaccactcagaaatatttttcatccacaaagcaggaaaaacataaaatcatttacatttcacattggcaccaaaaaggttaactgccctgccttcttggattagaaaaactaaagctgagtgataagtagttttgcaggcgtttgaacatgcctaagcctttaaatcagcaaaatactttctaaaaattctgattacaaaagtaatacatacttataaaaaattcgaacagaacaaaatgaaaaaagtagaaagtgaaaaggcccctataaaacccctctggggcccctcccccaatccccccctccccgaagagaaaccacatttaacagtttggtgtatatctttccaaatcttttgttctatgcatattaaaaacatacatactttgatctggctcagactatacatagtgttttgccacttgcattttacacttaacatatctttgacatctttccatgtcagtacatgttggctcgatagtattctatcattaaatacgctttcaaaaatggcaaatcactttaaaaaaataattcgcacaagtacgtgtttataactttaaaagaaaatggacagaatcctaaaacacaacaaccaacctctaaaaacaatctctatctttccaccagcatggaacaatttattcctttttcacacaaaacaaattatgtgattggggagattaactctaatctccacatttatatacagaaagctccatttgttaagcctatctgaaaagaataaaaaatccagatgattaattcacttacacttagaaattaaatcagtatactatgaatacacattgtgttcagttatagtatgatgcttcttattcttagtctatggtttcaattaaataacagtaaaaaaaatggataatacagctaataccctgaaaaatcaagaaattcaaagattatattgccaactaaaacactgccatgtacattttttttcctacttggtagcaaatgctaatggaattcaatcctgattacttaaagtcagttcacatcacacattcaatcagggtaataagaacaacataacatgcctactatagagttagattaagacataaaaattttttgcttgaaagtaatgactgtgtagcacatgggacacttgtcaactgcttcagcacattgtttacaagtgactagatgtccacaaggaacaaaaacgatagcaatatttctatccatacagattttgcaaagcttctcctcttgcaggcgccttagctgctcttcagtactaatctctttctgtaatgaagtctgacttgactcatcttgcatactgtctttctgagcattcactagatctgcaaccagaacctcaagtgatttatagttgctcccagatatctgaattttttcctccattattttcttaatgtccttgaaactgaaccccattcgtatagcttcttgtaccataggattttggaagatggtatcatcaattcttctagttagtgatggtgttttctcagtagttcttaccagacactcctcaagtgaatgagttaaatgaatattgtttatatattcttgtcccttctgttctaacagatatttgcaccctggataccatttagcatgttgttcccaagggtcttcactgggcttccaatcagttagccctcctccacagtgaaagcactttactttatcaccttcacctaaagcataaaatccagctcttgcaagctgctccttgttaactgagtatatccatgtcccaaaagtaaagatccgtgcttcataatctgccatggatggatttcttggaagatttgttgaatttgggaaattcctatcagaactcacagcatcagattcacttcgaatattaagattccggcccaaaacaaagaagcaattaggaaagtgtcgcctgtgttctgaccaggcacgatcacaaggttcccaatttttcagttttccaccacaacaaaagcactgcacttggtcaccaatacctgtgtagtagagtccagcacttgctaactctcttggggttaggtgagcatagtctggccagttctgaaaggactttaatctagcttcttcactatacatggcagggttcctcgggtatatggtgtctgatatatctacaacctgcccagttctcaaaagatagtctgcatgtgtctcagatggcctgtctaaggcaaaatgatctctgcttcccagatagttttcaactttgtactgaccattctggataccagaatttgtagactgcgtggcactattttcaagataaaagccgttgataaatctgcaatttggggatactttcctgtgtcttccaactgctgagtctccatattgccatctatctacagctgcatgacaactaaagcaccgcacggtatctccttcaccagtataaagaaaccctgctcgtgccagtgttgatgctgaaacaggactaccacttggaaaattagcaaaagtttttaatctattaaactcttctacaaattcttcttccttattgatgtctgcaggtacacaagttttagatccttcaaaactgttaaaagtcatcttctcttgaaaataggacttgtccaccttttcgcgccaggacagccggcccgaactgccccgcggcgatcggctcggtccaaggggagggtcccggaggaggcgcggcccgagccccaatctggaaatgccaactccgctctgcggcttggccccagccacttgggccgggcgtccctcgatgagcgccacgccggctccgggcgccgccaaggtcccgccacctccccgaaccggatgggggcagtaag

SEQ ID NO: 14253 - RNA, 5816 nt, Homo sapiens
  source 1..5816: mol_type = other RNA
gctgggattacaggcatgagccaccgcgcccagctgatttatatcttatctatgagaaacaccaaaaactatgagtaagcatcactgagttatcatgtaagaattttttctaagttttagcccaaatttccaggtcaagacaaacccacagagaggtaaaagggtattaggatgggagttcatatttacagcaggaactttacatacatggtctccttgagctcttgcaaccttgtaagataagtattattttcctttcacagatgaataaactgctaccctttttttaacaagtagatttgactaaaaagaactatgtcaaatattgcttcccattttcttatttcttttttttttttttttgagacagagtcttgctctgttgcccaggctggagtgcagtggcgagatctcggctcactgcaagctctgcctcccgggttcacaccattctcctgcctcagcctcccgagtagctgggactacaggcgcccgccaccacgcccggctaattttctgttttttagtagagacggggtttcaccgtgttagccaggatggtctcgatctcctgacctcgtgatccacctgcctcagcctcccaaagtgctgggattacaggcgtgagccactgagcccagccccattttatttcatttctctaacagcaatgatatatatacatcccatagtatatcctactgatatactagcccctttccccattcaacacctgtgtaatcaggaaataaaacaatgattcgggtttaaagggtatatcatgtgaaactaatgctggggcggtagtctccattcatagttcaaaatacaaattttatccactaaaatggaaacacaaaaaacaactactgaaatgtaaataatataacaacaaaaataacaaaatatcataatacacagggccaaatcacattatatacactcactacacccactctaccctaccttagcccgtaatcaaagggacaggggaaaaaaccaaatgtagcaggaaaggcaatataaagctattaattaattaactggaatttagtttgtaaatgctaaaaccagttctcaaaaattaagacaatgcttttgatcagcagactaaattattacaaataaagataagtacttattgcaaaactacttgaatctttgcatgactaaaatgtaaaataagtggtgacttgaaatcctagagtgaactttatacagaaaaggaatagtctacatgtagacactgagaactcttgggagggggaaaagatttggatatggctatagttttgactttgcaaatgatcaatttttgcggaattagatggaaaagatccggtgctttttatagttcaaacacagacaaatgctgttaagtctccaaaaatttgattagaagttggagtgctgagtgattttaagaacctgaagcaacagcatttctaaacaattcttaaaataaacttgttagccacatcagcgttgtgcattaaatttcacaactcatggagaggaagaaaaaaagtcttgcttaactctaaacatacaagttttagaagaattttaatgaagtgcggctcccagaacaggaaaagccttatgttaaaacaattcagtccttgagtccttggctaacaactagattgaactacctacctgacttggaagtgaagtgtcctggaaaacatattttaaaaattttaacacttttctccccttgtagaaaactttaaatttaaagtctagactatacagaccaaattcaagttaatgactatataaccaaactaagtggcagacagtgcaaaggtgaagaactgaggatttacatactaaaacagaaacagggcagtcattatttaatttttaaaactctcatttaaatttgcaatgttttagccgggcgtggtggctcaagcctgtaatcccagcactttgggagggcaaggcgagtggatctcttgaggtcaggagtttgataccagcctggccaacatggtgaaaccccgtctctactaaaaataaaaaaaaattagtcgggcatggtggcacctgcctgtaattccagctactcaggaagctgaggcacgagaatcgcttgaacccagaaggcggaggttgcagtgagcagagatcactccactgcactccagcctgggtgacaagcaagactccatctcaaaaagaaaattaaataaataaaataaatttgcaatgttttaaatgaatatcacttaaagtagtaatcaacagaagttaggagaacataacaatactctttctcttagaaagtacaacaaaaatataattttttacagttttactctcaaactttcctctgtagtaacatgccttactcacctctacaataggtttgttgtgagaatcttgtaatgtaaaccctggacgttctatgaagcatttttaaacttctagtttataccctactgattcttattcaagtgttttttaaaaaatatttaaacaactattcttcttttcttgccaatatttttataatttccaagaggttttaaggatcttgagagaacatttatttcagaagtatctactactattactagccaagaaaacaaatgtaggtagaggaaagacttaacattttgtcctatatacatcttaatcatcctaacggtaaaaactcacatgaaactttaagatacaagatgatatgagaatctcaacatggaaagctgtcactataactacaagcagtgtacaaacatgcttctacttttacctacataagctgacagatgtttaaaatactgagttaacaaagatcttttagtaaagtgacttaggcaggcttaaactagcaaggattaaggatgaatccttactaattaattggaagatctgagacatattttatatttcattttacaaaatcagaaatacttattttgaaacaagataagacatggtctacctgtcaaaaaactaccactcagaaatatttttcatccacaaagcaggaaaaacataaaatcatttacatttcacattggcaccaaaaaggttaactgccctgccttcttggattagaaaaactaaagctgagtgataagtagttttgcaggcgtttgaacatgcctaagcctttaaatcagcaaaatactttctaaaaattctgattacaaaagtaatacatacttataaaaaattcgaacagaacaaaatgaaaaaagtagaaagtgaaaaggcccctataaaacccctctggggcccctcccccaatccccccctccccgaagagaaaccacatttaacagtttggtgtatatctttccaaatcttttgttctatgcatattaaaaacatacatactttgatctggctcagactatacatagtgttttgccacttgcattttacacttaacatatctttgacatctttccatgtcagtacatgttggctcgatagtattctatcattaaatacgctttcaaaaatggcaaatcactttaaaaaaataattcgcacaagtacgtgtttataactttaaaagaaaatggacagaatcctaaaacacaacaaccaacctctaaaaacaatctctatctttccaccagcatggaacaatttattcctttttcacacaaaacaaattatgtgattggggagattaactctaatctccacatttatatacagaaagctccatttgttaagcctatctgaaaagaataaaaaatccagatgattaattcacttacacttagaaattaaatcagtatactatgaatacacattgtgttcagttatagtatgatgcttcttattcttagtctatggtttcaattaaataacagtaaaaaaaatggataatacagctaataccctgaaaaatcaagaaattcaaagattatattgccaactaaaacactgccatgtacattttttttcctacttggtagcaaatgctaatggaattcaatcctgattacttaaagtcagttcacatcacacattcaatcagggtaataagaacaacataacatgcctactatagagttagattaagacataaaaattttttgcttgaaagtaatgactgtgtagcacatgggacacttgtcaactgcttcagcacattgtttacaagtgactagatgtccacaaggaacaaaaacgatagcaatatttctatccatacagattttgcaaagcttctcctcttgcaggcgccttagctgctcttcagtactaatctctttctgtaatgaagtctgacttgactcatcttgcatactgtctttctgagcattcactagatctgcaaccagaacctcaagtgatttatagttgctcccagatatctgaattttttcctccattattttcttaatgtccttgaaactgaaccccattcgtatagcttcttgtaccataggattttggaagatggtatcatcaattcttctagttagtgatggtgttttctcagtagttcttaccagacactcctcaagtgaatgagttaaatgaatattgtttatatattcttgtcccttctgttctaacagatatttgcaccctggataccatttagcatgttgttcccaagggtcttcactgggcttccaatcagttagccctcctccacagtgaaagcactttactttatcaccttcacctaaagcataaaatccagctcttgcaagctgctccttgttaactgagtatatccatgtcccaaaagtaaagatccgtgcttcataatctgccatggatggatttcttggaagatttgttgaatttgggaaattcctatcagaactcacagcatcagattcacttcgaatattaagattccggcccaaaacaaagaagcaattaggaaagtgtcgcctgtgttctgaccaggcacgatcacaaggttcccaatttttcagttttccaccacaacaaaagcactgcacttggtcaccaatacctgtgtagtagagtccagcacttgctaactctcttggggttaggtgagcatagtctggccagttctgaaaggactttaatctagcttcttcactatacatggcagggttcctcgggtatatggtgtctgatatatctacaacctgcccagttctcaaaagatagtctgcatgtgtctcagatggcctgtctaaggcaaaatgatctctgcttcccagatagttttcaactttgtactgaccattctggataccagaatttgtagactgcgtggcactattttcaagataaaagccgttgataaatctgcaatttggggatactttcctgtgtcttccaactgctgagtctccatattgccatctatctacagctgcatgacaactaaagcaccgcacggtatctccttcaccagtataaagaaaccctgctcgtgccagtgttgatgctgaaacaggactaccacttggaaaattagcaaaagtttttaatctattaaactcttctacaaattcttcttccttattgatgtctgcaggtacacaagttttagatccttcaaaactgttaaaagtcatcttctcttgaaaataggacttgtccaccttttcgcgccaggacagccggcccgaactgccccgcggcgatcggctcggtccaaggggagggtcccggaggaggcgcggcccgagccccaatctggaaatgccaactccgctctgcggcttggccccagcctaggtgaaggaaacggaagtcccttcgtctccctcacgcgcctctaccggccggcccatcccctggagaaacccggagtcgtgaaacccgaagtgtgtccacgtcagggcctc

SEQ ID NO: 14254 - RNA, 5606 nt, Homo sapiens
  source 1..5606: mol_type = other RNA
gctgggattacaggcatgagccaccgcgcccagctgatttatatcttatctatgagaaacaccaaaaactatgagtaagcatcactgagttatcatgtaagaattttttctaagttttagcccaaatttccaggtcaagacaaacccacagagaggtaaaagggtattaggatgggagttcatatttacagcaggaactttacatacatggtctccttgagctcttgcaaccttgtaagataagtattattttcctttcacagatgaataaactgctaccctttttttaacaagtagatttgactaaaaagaactatgtcaaatattgcttcccattttcttatttcttttttttttttttttgagacagagtcttgctctgttgcccaggctggagtgcagtggcgagatctcggctcactgcaagctctgcctcccgggttcacaccattctcctgcctcagcctcccgagtagctgggactacaggcgcccgccaccacgcccggctaattttctgttttttagtagagacggggtttcaccgtgttagccaggatggtctcgatctcctgacctcgtgatccacctgcctcagcctcccaaagtgctgggattacaggcgtgagccactgagcccagccccattttatttcatttctctaacagcaatgatatatatacatcccatagtatatcctactgatatactagcccctttccccattcaacacctgtgtaatcaggaaataaaacaatgattcgggtttaaagggtatatcatgtgaaactaatgctggggcggtagtctccattcatagttcaaaatacaaattttatccactaaaatggaaacacaaaaaacaactactgaaatgtaaataatataacaacaaaaataacaaaatatcataatacacagggccaaatcacattatatacactcactacacccactctaccctaccttagcccgtaatcaaagggacaggggaaaaaaccaaatgtagcaggaaaggcaatataaagctattaattaattaactggaatttagtttgtaaatgctaaaaccagttctcaaaaattaagacaatgcttttgatcagcagactaaattattacaaataaagataagtacttattgcaaaactacttgaatctttgcatgactaaaatgtaaaataagtggtgacttgaaatcctagagtgaactttatacagaaaaggaatagtctacatgtagacactgagaactcttgggagggggaaaagatttggatatggctatagttttgactttgcaaatgatcaatttttgcggaattagatggaaaagatccggtgctttttatagttcaaacacagacaaatgctgttaagtctccaaaaatttgattagaagttggagtgctgagtgattttaagaacctgaagcaacagcatttctaaacaattcttaaaataaacttgttagccacatcagcgttgtgcattaaatttcacaactcatggagaggaagaaaaaaagtcttgcttaactctaaacatacaagttttagaagaattttaatgaagtgcggctcccagaacaggaaaagccttatgttaaaacaattcagtccttgagtccttggctaacaactagattgaactacctacctgacttggaagtgaagtgtcctggaaaacatattttaaaaattttaacacttttctccccttgtagaaaactttaaatttaaagtctagactatacagaccaaattcaagttaatgactatataaccaaactaagtggcagacagtgcaaaggtgaagaactgaggatttacatactaaaacagaaacagggcagtcattatttaatttttaaaactctcatttaaatttgcaatgttttagccgggcgtggtggctcaagcctgtaatcccagcactttgggagggcaaggcgagtggatctcttgaggtcaggagtttgataccagcctggccaacatggtgaaaccccgtctctactaaaaataaaaaaaaattagtcgggcatggtggcacctgcctgtaattccagctactcaggaagctgaggcacgagaatcgcttgaacccagaaggcggaggttgcagtgagcagagatcactccactgcactccagcctgggtgacaagcaagactccatctcaaaaagaaaattaaataaataaaataaatttgcaatgttttaaatgaatatcacttaaagtagtaatcaacagaagttaggagaacataacaatactctttctcttagaaagtacaacaaaaatataattttttacagttttactctcaaactttcctctgtagtaacatgccttactcacctctacaataggtttgttgtgagaatcttgtaatgtaaaccctggacgttctatgaagcatttttaaacttctagtttataccctactgattcttattcaagtgttttttaaaaaatatttaaacaactattcttcttttcttgccaatatttttataatttccaagaggttttaaggatcttgagagaacatttatttcagaagtatctactactattactagccaagaaaacaaatgtaggtagaggaaagacttaacattttgtcctatatacatcttaatcatcctaacggtaaaaactcacatgaaactttaagatacaagatgatatgagaatctcaacatggaaagctgtcactataactacaagcagtgtacaaacatgcttctacttttacctacataagctgacagatgtttaaaatactgagttaacaaagatcttttagtaaagtgacttaggcaggcttaaactagcaaggattaaggatgaatccttactaattaattggaagatctgagacatattttatatttcattttacaaaatcagaaatacttattttgaaacaagataagacatggtctacctgtcaaaaaactaccactcagaaatatttttcatccacaaagcaggaaaaacataaaatcatttacatttcacattggcaccaaaaaggttaactgccctgccttcttggattagaaaaactaaagctgagtgataagtagttttgcaggcgtttgaacatgcctaagcctttaaatcagcaaaatactttctaaaaattctgattacaaaagtaatacatacttataaaaaattcgaacagaacaaaatgaaaaaagtagaaagtgaaaaggcccctataaaacccctctggggcccctcccccaatccccccctccccgaagagaaaccacatttaacagtttggtgtatatctttccaaatcttttgttctatgcatattaaaaacatacatactttgatctggctcagactatacatagtgttttgccacttgcattttacacttaacatatctttgacatctttccatgtcagtacatgttggctcgatagtattctatcattaaatacgctttcaaaaatggcaaatcactttaaaaaaataattcgcacaagtacgtgtttataactttaaaagaaaatggacagaatcctaaaacacaacaaccaacctctaaaaacaatctctatctttccaccagcatggaacaatttattcctttttcacacaaaacaaattatgtgattggggagattaactctaatctccacatttatatacagaaagctccatttgttaagcctatctgaaaagaataaaaaatccagatgattaattcacttacacttagaaattaaatcagtatactatgaatacacattgtgttcagttatagtatgatgcttcttattcttagtctatggtttcaattaaataacagtaaaaaaaatggataatacagctaataccctgaaaaatcaagaaattcaaagattatattgccaactaaaacactgccatgtacattttttttcctacttggtagcaaatgctaatggaattcaatcctgattacttaaagtcagttcacatcacacattcaatcagggtaataagaacaacataacatgcctactatagagttagattaagacataaaaattttttgcttgaaagtaatgactgtgtagcacatgggacacttgtcaactgcttcagcacattgtttacaagtgactagatgtccacaaggaacaaaaacgatagcaatatttctatccatacagattttgcaaagcttctcctcttgcaggcgccttagctgctcttcagtactaatctctttctgtaatgaagtctgacttgactcatcttgcatactgtctttctgagcattcactagatctgcaaccagaacctcaagtgatttatagttgctcccagatatctgaattttttcctccattattttcttaatgtccttgaaactgaaccccattcgtatagcttcttgtaccataggattttggaagatggtatcatcaattcttctagttagtgatggtgttttctcagtagttcttaccagacactcctcaagtgaatgagttaaatgaatattgtttatatattcttgtcccttctgttctaacagatatttgcaccctggataccatttagcatgttgttcccaagggtcttcactgggcttccaatcagttagccctcctccacagtgaaagcactttactttatcaccttcacctaaagcataaaatccagctcttgcaagctgctccttgttaactgagtatatccatgtcccaaaagtaaagatccgtgcttcataatctgccatggatggatttcttggaagatttgttgaatttgggaaattcctatcagaactcacagcatcagattcacttcgaatattaagattccggcccaaaacaaagaagcaattaggaaagtgtcgcctgtgttctgaccaggcacgatcacaaggttcccaatttttcagttttccaccacaacaaaagcactgcacttggtcaccaatacctgtgtagtagagtccagcacttgctaactctcttggggttaggtgagcatagtctggccagttctgaaaggactttaatctagcttcttcactatacatggcagggttcctcgggtatatggtgtctgatatatctacaacctgcccagttctcaaaagatagtctgcatgtgtctcagatggcctgtctaaggcaaaatgatctctgcttcccagatagttttcaactttgtactgaccattctggataccagaatttgtagactgcgtggcactattttcaagataaaagccgttgataaatctgcaatttggggatactttcctgtgtcttccaactgctgagtctccatattgccatctatctacagctgcatgacaactaaagcaccgcacggtatctccttcaccagtataaagaaaccctgctcgtgccagtgttgatgctgaaacaggactaccacttggaaaattagcaaaagtttttaatctattaaactcttctacaaattcttcttccttattgatgtctgcaggtacacaagttttagatccttcaaaactgttaaaagtcatcttctcttgaaaataggacttgtccaccttttctagcgcgcgcacatgcgcagtgagcacctc

SEQ ID NO: 14255 - RNA, 5671 nt, Homo sapiens
  source 1..5671: mol_type = other RNA
gctgggattacaggcatgagccaccgcgcccagctgatttatatcttatctatgagaaacaccaaaaactatgagtaagcatcactgagttatcatgtaagaattttttctaagttttagcccaaatttccaggtcaagacaaacccacagagaggtaaaagggtattaggatgggagttcatatttacagcaggaactttacatacatggtctccttgagctcttgcaaccttgtaagataagtattattttcctttcacagatgaataaactgctaccctttttttaacaagtagatttgactaaaaagaactatgtcaaatattgcttcccattttcttatttcttttttttttttttttgagacagagtcttgctctgttgcccaggctggagtgcagtggcgagatctcggctcactgcaagctctgcctcccgggttcacaccattctcctgcctcagcctcccgagtagctgggactacaggcgcccgccaccacgcccggctaattttctgttttttagtagagacggggtttcaccgtgttagccaggatggtctcgatctcctgacctcgtgatccacctgcctcagcctcccaaagtgctgggattacaggcgtgagccactgagcccagccccattttatttcatttctctaacagcaatgatatatatacatcccatagtatatcctactgatatactagcccctttccccattcaacacctgtgtaatcaggaaataaaacaatgattcgggtttaaagggtatatcatgtgaaactaatgctggggcggtagtctccattcatagttcaaaatacaaattttatccactaaaatggaaacacaaaaaacaactactgaaatgtaaataatataacaacaaaaataacaaaatatcataatacacagggccaaatcacattatatacactcactacacccactctaccctaccttagcccgtaatcaaagggacaggggaaaaaaccaaatgtagcaggaaaggcaatataaagctattaattaattaactggaatttagtttgtaaatgctaaaaccagttctcaaaaattaagacaatgcttttgatcagcagactaaattattacaaataaagataagtacttattgcaaaactacttgaatctttgcatgactaaaatgtaaaataagtggtgacttgaaatcctagagtgaactttatacagaaaaggaatagtctacatgtagacactgagaactcttgggagggggaaaagatttggatatggctatagttttgactttgcaaatgatcaatttttgcggaattagatggaaaagatccggtgctttttatagttcaaacacagacaaatgctgttaagtctccaaaaatttgattagaagttggagtgctgagtgattttaagaacctgaagcaacagcatttctaaacaattcttaaaataaacttgttagccacatcagcgttgtgcattaaatttcacaactcatggagaggaagaaaaaaagtcttgcttaactctaaacatacaagttttagaagaattttaatgaagtgcggctcccagaacaggaaaagccttatgttaaaacaattcagtccttgagtccttggctaacaactagattgaactacctacctgacttggaagtgaagtgtcctggaaaacatattttaaaaattttaacacttttctccccttgtagaaaactttaaatttaaagtctagactatacagaccaaattcaagttaatgactatataaccaaactaagtggcagacagtgcaaaggtgaagaactgaggatttacatactaaaacagaaacagggcagtcattatttaatttttaaaactctcatttaaatttgcaatgttttagccgggcgtggtggctcaagcctgtaatcccagcactttgggagggcaaggcgagtggatctcttgaggtcaggagtttgataccagcctggccaacatggtgaaaccccgtctctactaaaaataaaaaaaaattagtcgggcatggtggcacctgcctgtaattccagctactcaggaagctgaggcacgagaatcgcttgaacccagaaggcggaggttgcagtgagcagagatcactccactgcactccagcctgggtgacaagcaagactccatctcaaaaagaaaattaaataaataaaataaatttgcaatgttttaaatgaatatcacttaaagtagtaatcaacagaagttaggagaacataacaatactctttctcttagaaagtacaacaaaaatataattttttacagttttactctcaaactttcctctgtagtaacatgccttactcacctctacaataggtttgttgtgagaatcttgtaatgtaaaccctggacgttctatgaagcatttttaaacttctagtttataccctactgattcttattcaagtgttttttaaaaaatatttaaacaactattcttcttttcttgccaatatttttataatttccaagaggttttaaggatcttgagagaacatttatttcagaagtatctactactattactagccaagaaaacaaatgtaggtagaggaaagacttaacattttgtcctatatacatcttaatcatcctaacggtaaaaactcacatgaaactttaagatacaagatgatatgagaatctcaacatggaaagctgtcactataactacaagcagtgtacaaacatgcttctacttttacctacataagctgacagatgtttaaaatactgagttaacaaagatcttttagtaaagtgacttaggcaggcttaaactagcaaggattaaggatgaatccttactaattaattggaagatctgagacatattttatatttcattttacaaaatcagaaatacttattttgaaacaagataagacatggtctacctgtcaaaaaactaccactcagaaatatttttcatccacaaagcaggaaaaacataaaatcatttacatttcacattggcaccaaaaaggttaactgccctgccttcttggattagaaaaactaaagctgagtgataagtagttttgcaggcgtttgaacatgcctaagcctttaaatcagcaaaatactttctaaaaattctgattacaaaagtaatacatacttataaaaaattcgaacagaacaaaatgaaaaaagtagaaagtgaaaaggcccctataaaacccctctggggcccctcccccaatccccccctccccgaagagaaaccacatttaacagtttggtgtatatctttccaaatcttttgttctatgcatattaaaaacatacatactttgatctggctcagactatacatagtgttttgccacttgcattttacacttaacatatctttgacatctttccatgtcagtacatgttggctcgatagtattctatcattaaatacgctttcaaaaatggcaaatcactttaaaaaaataattcgcacaagtacgtgtttataactttaaaagaaaatggacagaatcctaaaacacaacaaccaacctctaaaaacaatctctatctttccaccagcatggaacaatttattcctttttcacacaaaacaaattatgtgattggggagattaactctaatctccacatttatatacagaaagctccatttgttaagcctatctgaaaagaataaaaaatccagatgattaattcacttacacttagaaattaaatcagtatactatgaatacacattgtgttcagttatagtatgatgcttcttattcttagtctatggtttcaattaaataacagtaaaaaaaatggataatacagctaataccctgaaaaatcaagaaattcaaagattatattgccaactaaaacactgccatgtacattttttttcctacttggtagcaaatgctaatggaattcaatcctgattacttaaagtcagttcacatcacacattcaatcagggtaataagaacaacataacatgcctactatagagttagattaagacataaaaattttttgcttgaaagtaatgactgtgtagcacatgggacacttgtcaactgcttcagcacattgtttacaagtgactagatgtccacaaggaacaaaaacgatagcaatatttctatccatacagattttgcaaagcttctcctcttgcaggcgccttagctgctcttcagtactaatctctttctgtaatgaagtctgacttgactcatcttgcatactgtctttctgagcattcactagatctgcaaccagaacctcaagtgatttatagttgctcccagatatctgaattttttcctccattattttcttaatgtccttgaaactgaaccccattcgtatagcttcttgtaccataggattttggaagatggtatcatcaattcttctagttagtgatggtgttttctcagtagttcttaccagacactcctcaagtgaatgagttaaatgaatattgtttatatattcttgtcccttctgttctaacagatatttgcaccctggataccatttagcatgttgttcccaagggtcttcactgggcttccaatcagttagccctcctccacagtgaaagcactttactttatcaccttcacctaaagcataaaatccagctcttgcaagctgctccttgttaactgagtatatccatgtcccaaaagtaaagatccgtgcttcataatctgccatggatggatttcttggaagatttgttgaatttgggaaattcctatcagaactcacagcatcagattcacttcgaatattaagattccggcccaaaacaaagaagcaattaggaaagtgtcgcctgtgttctgaccaggcacgatcacaaggttcccaatttttcagttttccaccacaacaaaagcactgcacttggtcaccaatacctgtgtagtagagtccagcacttgctaactctcttggggttaggtgagcatagtctggccagttctgaaaggactttaatctagcttcttcactatacatggcagggttcctcgggtatatggtgtctgatatatctacaacctgcccagttctcaaaagatagtctgcatgtgtctcagatggcctgtctaaggcaaaatgatctctgcttcccagatagttttcaactttgtactgaccattctggataccagaatttgtagactgcgtggcactattttcaagataaaagccgttgataaatctgcaatttggggatactttcctgtgtcttccaactgctgagtctccatattgccatctatctacagctgcatgacaactaaagcaccgcacggtatctccttcaccagtataaagaaaccctgctcgtgccagtgttgatgctgaaacaggactaccacttggaaaattagcaaaagtttttaatctattaaactcttctacaaattcttcttccttattgatgtctgcaggtacacaagttttagatccttcaaaactgttaaaagtcatcttctcttgaaaataggacttgtccaccttttcttaggtgtcacagggtttaggaaggcaatcctgcaggcctgaagtcacccacccacccacgcctgccgtcggcagtccgaggaacccgggcaagc

SEQ ID NO: 14256 - RNA, 8858 nt, Homo sapiens
  source 1..8858: mol_type = other RNA
gctgggattacaggcatgagccaccgcgcccagtccggtttattcattttctgtgtcctaatatcttcattaagttaatttccagtacagttgtacctcagtatctgcagggagttggttccaggatccctttgactatcaaaatccacagatgctcaagggccctatataaaatggtgtcttttctggtgttttttgtttttgttttttgagacaaggtctcattctgttgccaggctggagagcagtggctcagtcacagctcactgtagcctcgacctcctgggctcaggtgattctcccacctcaacctaccaagtagctgggactataggcacgtgccactatgcctggtcaatttttgtattttgtgtagacagggttttgccatgttgcccaggctggtctacaactcctgggctcaagcagtctgcccacctccatcccccaaaaacgttgggattacacgtgtgagccaccatgccaggcctggagtagtatttgcatgtaacctatgcacatcctcccatatactttaagtcatctctggattacttataatatctaatacaatataaatactatgtaaatagttgttacactgtattttaaaatatgtatatttttattgttgtattattttttcaaatctttcccatcacattagttgattctgaagatgcagagcccgtaaatatggacggccaactatgttgtatttctcatttctgaaaattctatttagtttctaaagtttgtttccttcttctaaatatatttaaatatactttatttgtagcctctgcttaataattctattatctaaagtccttgggggtttaaatcttattgccttctgactcttatgataaattgtttccttgcatgttctattattttgaattgtgatctcaacttcattggggtttcatatgtggatatcctgttaggtctgagttaacatgcaacaatctagaaattctgtttccttctggcaactgccctagaaatacttttcatattaagttcacaggattcgcagaccacacaggtagtataaatttgaatcccaaactggtgaaaaggtaggtctatggtgacaaattcccaggaatgacttttattctctgtaccatgagtccaagctaacacaagcactagagggtggattttgttttttaatccttccattgagggtgaatgtctttaaaggtcctggctttgtatgtggatctcaatccaacttctcaccttgtaggggggcctaagactttacctcgagtgtccttgcgtgacctttaaaacccgagcatactggttacagaaactagggactgtctttacgcccaggcagtcacaaagcataaaccacacaccatactgttgttaaatttcctgtttagggctccgcccaggctggaatgcaatggcatgatctcagctcactgcaacctccatctcccaggttcaaatgattctgcctcagcctcccaagtagctgggattaccggcatgcgccaccatgcccagctaatttttatatttttagaagagatggattttcaccatgttggccaggctagtctcaaactcctgacctcaagtgatccgcctgcctcagcctcccaaagtgctgggattacaggcgtgagccaccaggcctggcggaaccttgatcttttaaatgtgaatttcagatatttctattacctgtaaggagagaggtggggaagacgaaggttgaagggaatattgaataaataactcctgtgtactagccctcaatacatgagatatttgataacagctatacaaaacaagccatgttaatagatgagaaattaaagctcagaaaggtcaaataatttcgctaaggtcacaatgtactattacacccgaattcacgttggaattaactagtcagatccattttcattctggacatggtggtgtatgcctgtagtcccagctatttgggggcctgaagtgagaggactgcttgtgcctaggaattcatgtacagcctgggcaacatagcaagaaactgcttctaaaaataaataggctgggtgcagtggctcacgcctgtaatcccagcactttgggaggtggaggcaggtggatcacttgaggtcaggagttcaagaccagcctggccaacacggcgaaaccccatctctactaaaaatacaaaaaattagctgggtgtggtggtgcgtgcctgtaatcccagttacttgggaggctgaggcaggagaagagctttaacccaggaagcagaggttgtggtgagctgagatcacgtcactgcactccagcctgggcaacagagcaagactctgtctcaaataaaaataaataactttgggaggccgaagtgggaggatcccgaggtcgagatcgagaccatcctggctaacacagtgaaaccccatctctactaaaaatacaaaaaattagctgggcatggtggcaggcacctgtagtctcccagctacttggaaggctgaggcagaagaattgcttgaacctgggaggcggaggttgcagtgagccgagatcgtgccactgcattccagcctgggcaacagagagagactccatctcaaaaaattaaaaataagttaacaaataatcaattttcttcctctacagcagaggtcagcaaacttattctgttaaaggccaaacagtaaatattttaggcctcataagccatatggtattggctgcaactattcagttttactgttgtatcattaaagcagccactgaaaagtgtaaacaaatgagcatgactgtgttcccataaaactttaaggacattgacatttgaatttcataaaattttcacatataacaatactattattacttggatcttttccccaaccatataaaaatttaaaacccgttgctaatgcatgggtcttacaaaaacagcctggagttgacccacgggccgtggtttgctgacccttatcatacaccataacacctccttggaagtacacctctctaatgcctttgttccaaacaatactgggttaggaaagacatggaaaaaggaaaatgagatacattattttttgtaccctatgggggattgaggggttgttgctacatagccccctcaatttgtgctgtagcaatatgcagttaagatccttattctaatgttaaatgtctcttctgtggcttatcctaactttaaaaaaaaaaaaaagaagccatcttacgtaaatgaacttacaattttaagacagggtctcactctgtcacccaggctggagtgcagtggtacaatcacggctcattgcagcctcgacctctcaggctcgagagatcctcccaccccaacttcccaagtagctgggactacaggtgtgcaccactatgcctagctcatcttttttttttttttttttttcctttaaaagatatggagtctcgctattttgcccaggctggtcttgaactcctggactcaagcaatccacctgcctcagcctcccagagtgttgggattacaggtgtgagccactgtgcccggcctgaattatcttcttattgtaaaatttcctttaatgcttaatagttgatgtatattaagtgctaactaaatgttcactgataaacattaatcagatgctgctaaatattgtctttctttattcacagatgatagtcaatgggcacaacatataagtagttacaatgaaatgagaagcaatatagcagtcaggctatatgcatgatttaacaacaaaattatcacttccttttaatttagaataagggacaatttaaaaagcatctcttggccctatcatttctgttccagtagttagtgttcatatgtgaatactaagtttgacattcctttctcccatagaaccattttggtgatttggatggtggccactacactgctttctgcaagaattcagtcacccaggcctgatatagctttgataacacacgagtcagtgagattccagatacttctgttcaaaatgctatggatctcctgttctatagctgccagcccttttccataccaatacaaaagcgttaagagccaggaaaatggtgtttcctgaacactgcaaaacaagcagtcagcatctggtggtagagttttgcttggtcattaaactcttagaacttacttgcatcattaacatttttatgccttgtgggcatgttatacaacctttcatcttaagataaatctgtcgtccagaagatgggtcttggttcactaaaaaaggcagtgtgaatataatgcaatgctaatggatgcaggccttcaaaacactgcaattatatagtgagttcaggtttcaaaattcagtgtttatcagaaaatatctcataatcatatatattcaacaaattattttccaaagatactcatgaagctaaacaaaaataatttttgttcaaatggctcgatgagtttaagaatatgatttgaatatatttgatataataatttagccaagaagtggtctcttagactaattgtaaaacatgaaaagttgtcagcttcacaatttgaaccccatcctttcatcttctccctgagagcctgctaatggtggtctctttctgaagcacttttagaatcttatttttatatggagtgttttactgactatatatatagcaactgagtccctcggttaaataaattataagctcctttaaccctcttaatacatcactctgtaaagatgtagtttataatgcagttcactttgcaatcatgcctgactcccggcatttttactttaatatttagaatgaatattctcaatatgtgagaatactagtcttgaaagaatgactctgggtgttattatatagcacgtgtgtatataaaatctatggttttactgtcctatatttgataatacaatattaaagacagaacacccacagggttataaattatttttctcattaagattttaatgtagctgtaaatgaaattctcgttttaaaaaaattaaagtttccatttttttttttagaataaagatttagtgcacaaatacagcccaaagccaacagaaaaattgctttgccctgtcatttccctaagaaagcactgaagttaactcaaaataggctgaaagaaaaaaagcaatcctctgagttctaggtttcacaaaaggaccacgtgttaaactatgtacatcgatttgatgtgcaagtatgcaataaatatgtacacatacattcctatctgctttacatcattctagagtattcatagtatatcaagatgggatttagaaatgtgaaaaggccataacagtgaaaaggaaaaaaaaaagataacaatagtttttagaccagtcgaataataatgcttagctagttaattattttaactttggagcagactaaaaaagttgttttgaaataaatggtacctgtaagtgatgattactgcaatacttgttaaatgttatttgtcagcactgaccggaattatatagtgctagtaacacagctcccactgtcctagaattcctctaaatggccagctatagctaccattatcctgataagcatttcaagagttgtgttgctgagccttttaaaagataactagtttataacctatgtctccttatgtggctacatcagttactcgtggtcccaatgaagtataaaagaggatataagctgctgaagatttcacagaagaaacggagatatcagaaacttcatgatcatcaaacttaaaccaccgttgtcttgctgcatttttacaataggctgtgtagtggcctccatccagcccaccgtagtgatttgaaacagaaaacaaattatatttcttcaaattgttctttggaccaataacatactgtgacaagtcaagattttctaacgggaagtccacagatgtctgtaatttttgtttccacctgccatcgtaggaaaaacgtttcagatgcactaaaagcacaggtggtaacttccagatttctatcttttttagagaatcccgtcgagctctgcaatgactgcagtaaaatctgttgttatctgtgagtttttcttctttggaaaataatctaaggcaatcctgtaatgtacatttacttgtggatgctagtggtagagacaaatacatgaaggcctcaaatgtcctagactttttgtgacatgtgaggcactgtactgtagatttgaattgaccctgaaaaagtgcaacaataatagactcattgagctgcttgtgtttctgccaggcatgttctgcagctttaaagtcatcgagatgatcattattttcttctttatatctcttccgattatcagctttatttagatcttcatggagaccatccattaggaacagaagcaattcttgtgaatcttgctgactgtatcctgcaaactggtcattgatcttcccaatggtgattttaaagtcctttggactgatatatctatactgtcctgtccacagggctttcatgattataccaaattcttctgccacttcacctttatgccccaacaaatttgacctgttaatatcatcctgataacagtttcggttgaaataatcagccaaatgtggagcgttacataggcactgcaatattgagttcatataacaagtatttcctaagttacgaagtccagtaagagctggtccagaacctccaaaaacaggattgaggttccgaatctgagaagcagaaagccttgagatctcagctttaggataacatgttggcttgttttcccgattaactgttggagttactgttggcttcctcttctcttcctcttgaatagcctgggttatatctggggaggagtaggagcgcttcagtttggaaggttccctatcccgctcagcaggaatctgtggcttggctttatgagttggaggggtggaaggaggtgcagatgaaggagccatttccggtgggtacatatgaacagtgttggtgggtgaatgataataacgaaaggttccagtgattgggtcaagaaacttggcccagcctgaaggcagtcctggtacgatcctccccatttcttcacttcgtgctcttgtcaaaggttctcgttgagccttgcctgaacctgaatcccctgtcacagatgtatggggcacatctcctgttgactttttctgtatttctggggttggacaccttttccccctatcttctacagatttcttggcatcagaagtttcatgttcacttttactttgtctttttactcctgttatttctttgcccctctttgctgaggtttctttatcttctttcttggcctgttcactttctttcttctccatttcttcttttgctttttgttgcttctctgtaatttcattttcttcagcttcttgtttctttttggctttttgttcttgttcttccttcctcagtttctctttctgttcctcttgctgcctttcccgaagttctttttcttgtttgtttttttccattagaagagcagtttctgcatgaatacgagccttttcttcatctgttaacatgagagttggagaaaaaactactggcttggtggaacgatcaggaataacttttccactctgaggagattgttgctcatggtttgtactttcagattttattctatgctcttcaggcaatttgactgctggttttttagtacgatcaatctgtggaacattctttatactaggcactggctgaattatgggtgaaacatcagatttagaagcagcaactggttcaactggagttgatatattcagtggtcccattctctcattttgaccacttatcaattctatattttcatctacttctatagatgcaggtggcgtctgggcagcaggtttagaaggaattgattcttccaatgagggataagtaaaatccaatgagatagacacctcttcattctggcgtcgtgggggtggagtgaccttagcatttgttgtatactggggataacaaaggagccagttttcatagcctccctctaaaaccaaaggctcattgcgcaggacagttttactttcccacttgaaaagtgcatctttcagactccggagagttgttccaatctgtaaatctttggcagaactaaaccagtcaagaagtaccacatactccacattccccctcttcttccatgtgtctttagaatcatctggcaggtgtgcttcaatccaactagcagtgactcctggactgatggcttcttcaggaacactgagagaatgtaaaatacaggaatcctgataatcctgcattcttcgagcatccattataatcaagctgatgtttttatccgtcatcattgtgtatagttcctttgctgtgattgctcctttctctttggtctcacatttttcattcttttcaccattgctcttttgggttttgtctttggaatccaaaacattctccaaagagcctttagccaatgtgccaccatcctctcttcctgtttcctgccttttttgttgtagccgctgtgcttcctcctgcctgtctttttcctcaagttttttccggacttcagcttcttcatatctcttagtgcttattttctctggtttaacttctgtcttcttattaaggtcttttagtgaagaactgaggtagagttctttaggaactgaagccacagcaggcatgatgaattatctttacttttccactttcacaatggatgctatatttccttacaagtgcttctttccgtgacgccgggcgcgcttcactaacgccagccttctcgccaaatgcccatctcccaagaactcgagggagaattagccttggctaccaggacggaagccagcccagctc

SEQ ID NO: 14257 - RNA, 9176 nt, Homo sapiens
  source 1..9176: mol_type = other RNA
gctgggattacaggcatgagccaccgcgcccagtccggtttattcattttctgtgtcctaatatcttcattaagttaatttccagtacagttgtacctcagtatctgcagggagttggttccaggatccctttgactatcaaaatccacagatgctcaagggccctatataaaatggtgtcttttctggtgttttttgtttttgttttttgagacaaggtctcattctgttgccaggctggagagcagtggctcagtcacagctcactgtagcctcgacctcctgggctcaggtgattctcccacctcaacctaccaagtagctgggactataggcacgtgccactatgcctggtcaatttttgtattttgtgtagacagggttttgccatgttgcccaggctggtctacaactcctgggctcaagcagtctgcccacctccatcccccaaaaacgttgggattacacgtgtgagccaccatgccaggcctggagtagtatttgcatgtaacctatgcacatcctcccatatactttaagtcatctctggattacttataatatctaatacaatataaatactatgtaaatagttgttacactgtattttaaaatatgtatatttttattgttgtattattttttcaaatctttcccatcacattagttgattctgaagatgcagagcccgtaaatatggacggccaactatgttgtatttctcatttctgaaaattctatttagtttctaaagtttgtttccttcttctaaatatatttaaatatactttatttgtagcctctgcttaataattctattatctaaagtccttgggggtttaaatcttattgccttctgactcttatgataaattgtttccttgcatgttctattattttgaattgtgatctcaacttcattggggtttcatatgtggatatcctgttaggtctgagttaacatgcaacaatctagaaattctgtttccttctggcaactgccctagaaatacttttcatattaagttcacaggattcgcagaccacacaggtagtataaatttgaatcccaaactggtgaaaaggtaggtctatggtgacaaattcccaggaatgacttttattctctgtaccatgagtccaagctaacacaagcactagagggtggattttgttttttaatccttccattgagggtgaatgtctttaaaggtcctggctttgtatgtggatctcaatccaacttctcaccttgtaggggggcctaagactttacctcgagtgtccttgcgtgacctttaaaacccgagcatactggttacagaaactagggactgtctttacgcccaggcagtcacaaagcataaaccacacaccatactgttgttaaatttcctgtttagggctccgcccaggctggaatgcaatggcatgatctcagctcactgcaacctccatctcccaggttcaaatgattctgcctcagcctcccaagtagctgggattaccggcatgcgccaccatgcccagctaatttttatatttttagaagagatggattttcaccatgttggccaggctagtctcaaactcctgacctcaagtgatccgcctgcctcagcctcccaaagtgctgggattacaggcgtgagccaccaggcctggcggaaccttgatcttttaaatgtgaatttcagatatttctattacctgtaaggagagaggtggggaagacgaaggttgaagggaatattgaataaataactcctgtgtactagccctcaatacatgagatatttgataacagctatacaaaacaagccatgttaatagatgagaaattaaagctcagaaaggtcaaataatttcgctaaggtcacaatgtactattacacccgaattcacgttggaattaactagtcagatccattttcattctggacatggtggtgtatgcctgtagtcccagctatttgggggcctgaagtgagaggactgcttgtgcctaggaattcatgtacagcctgggcaacatagcaagaaactgcttctaaaaataaataggctgggtgcagtggctcacgcctgtaatcccagcactttgggaggtggaggcaggtggatcacttgaggtcaggagttcaagaccagcctggccaacacggcgaaaccccatctctactaaaaatacaaaaaattagctgggtgtggtggtgcgtgcctgtaatcccagttacttgggaggctgaggcaggagaagagctttaacccaggaagcagaggttgtggtgagctgagatcacgtcactgcactccagcctgggcaacagagcaagactctgtctcaaataaaaataaataactttgggaggccgaagtgggaggatcccgaggtcgagatcgagaccatcctggctaacacagtgaaaccccatctctactaaaaatacaaaaaattagctgggcatggtggcaggcacctgtagtctcccagctacttggaaggctgaggcagaagaattgcttgaacctgggaggcggaggttgcagtgagccgagatcgtgccactgcattccagcctgggcaacagagagagactccatctcaaaaaattaaaaataagttaacaaataatcaattttcttcctctacagcagaggtcagcaaacttattctgttaaaggccaaacagtaaatattttaggcctcataagccatatggtattggctgcaactattcagttttactgttgtatcattaaagcagccactgaaaagtgtaaacaaatgagcatgactgtgttcccataaaactttaaggacattgacatttgaatttcataaaattttcacatataacaatactattattacttggatcttttccccaaccatataaaaatttaaaacccgttgctaatgcatgggtcttacaaaaacagcctggagttgacccacgggccgtggtttgctgacccttatcatacaccataacacctccttggaagtacacctctctaatgcctttgttccaaacaatactgggttaggaaagacatggaaaaaggaaaatgagatacattattttttgtaccctatgggggattgaggggttgttgctacatagccccctcaatttgtgctgtagcaatatgcagttaagatccttattctaatgttaaatgtctcttctgtggcttatcctaactttaaaaaaaaaaaaaagaagccatcttacgtaaatgaacttacaattttaagacagggtctcactctgtcacccaggctggagtgcagtggtacaatcacggctcattgcagcctcgacctctcaggctcgagagatcctcccaccccaacttcccaagtagctgggactacaggtgtgcaccactatgcctagctcatcttttttttttttttttttttcctttaaaagatatggagtctcgctattttgcccaggctggtcttgaactcctggactcaagcaatccacctgcctcagcctcccagagtgttgggattacaggtgtgagccactgtgcccggcctgaattatcttcttattgtaaaatttcctttaatgcttaatagttgatgtatattaagtgctaactaaatgttcactgataaacattaatcagatgctgctaaatattgtctttctttattcacagatgatagtcaatgggcacaacatataagtagttacaatgaaatgagaagcaatatagcagtcaggctatatgcatgatttaacaacaaaattatcacttccttttaatttagaataagggacaatttaaaaagcatctcttggccctatcatttctgttccagtagttagtgttcatatgtgaatactaagtttgacattcctttctcccatagaaccattttggtgatttggatggtggccactacactgctttctgcaagaattcagtcacccaggcctgatatagctttgataacacacgagtcagtgagattccagatacttctgttcaaaatgctatggatctcctgttctatagctgccagcccttttccataccaatacaaaagcgttaagagccaggaaaatggtgtttcctgaacactgcaaaacaagcagtcagcatctggtggtagagttttgcttggtcattaaactcttagaacttacttgcatcattaacatttttatgccttgtgggcatgttatacaacctttcatcttaagataaatctgtcgtccagaagatgggtcttggttcactaaaaaaggcagtgtgaatataatgcaatgctaatggatgcaggccttcaaaacactgcaattatatagtgagttcaggtttcaaaattcagtgtttatcagaaaatatctcataatcatatatattcaacaaattattttccaaagatactcatgaagctaaacaaaaataatttttgttcaaatggctcgatgagtttaagaatatgatttgaatatatttgatataataatttagccaagaagtggtctcttagactaattgtaaaacatgaaaagttgtcagcttcacaatttgaaccccatcctttcatcttctccctgagagcctgctaatggtggtctctttctgaagcacttttagaatcttatttttatatggagtgttttactgactatatatatagcaactgagtccctcggttaaataaattataagctcctttaaccctcttaatacatcactctgtaaagatgtagtttataatgcagttcactttgcaatcatgcctgactcccggcatttttactttaatatttagaatgaatattctcaatatgtgagaatactagtcttgaaagaatgactctgggtgttattatatagcacgtgtgtatataaaatctatggttttactgtcctatatttgataatacaatattaaagacagaacacccacagggttataaattatttttctcattaagattttaatgtagctgtaaatgaaattctcgttttaaaaaaattaaagtttccatttttttttttagaataaagatttagtgcacaaatacagcccaaagccaacagaaaaattgctttgccctgtcatttccctaagaaagcactgaagttaactcaaaataggctgaaagaaaaaaagcaatcctctgagttctaggtttcacaaaaggaccacgtgttaaactatgtacatcgatttgatgtgcaagtatgcaataaatatgtacacatacattcctatctgctttacatcattctagagtattcatagtatatcaagatgggatttagaaatgtgaaaaggccataacagtgaaaaggaaaaaaaaaagataacaatagtttttagaccagtcgaataataatgcttagctagttaattattttaactttggagcagactaaaaaagttgttttgaaataaatggtacctgtaagtgatgattactgcaatacttgttaaatgttatttgtcagcactgaccggaattatatagtgctagtaacacagctcccactgtcctagaattcctctaaatggccagctatagctaccattatcctgataagcatttcaagagttgtgttgctgagccttttaaaagataactagtttataacctatgtctccttatgtggctacatcagttactcgtggtcccaatgaagtataaaagaggatataagctgctgaagatttcacagaagaaacggagatatcagaaacttcatgatcatcaaacttaaaccaccgttgtcttgctgcatttttacaataggctgtgtagtggcctccatccagcccaccgtagtgatttgaaacagaaaacaaattatatttcttcaaattgttctttggaccaataacatactgtgacaagtcaagattttctaacgggaagtccacagatgtctgtaatttttgtttccacctgccatcgtaggaaaaacgtttcagatgcactaaaagcacaggtggtaacttccagatttctatcttttttagagaatcccgtcgagctctgcaatgactgcagtaaaatctgttgttatctgtgagtttttcttctttggaaaataatctaaggcaatcctgtaatgtacatttacttgtggatgctagtggtagagacaaatacatgaaggcctcaaatgtcctagactttttgtgacatgtgaggcactgtactgtagatttgaattgaccctgaaaaagtgcaacaataatagactcattgagctgcttgtgtttctgccaggcatgttctgcagctttaaagtcatcgagatgatcattattttcttctttatatctcttccgattatcagctttatttagatcttcatggagaccatccattaggaacagaagcaattcttgtgaatcttgctgactgtatcctgcaaactggtcattgatcttcccaatggtgattttaaagtcctttggactgatatatctatactgtcctgtccacagggctttcatgattataccaaattcttctgccacttcacctttatgccccaacaaatttgacctgttaatatcatcctgataacagtttcggttgaaataatcagccaaatgtggagcgttacataggcactgcaatattgagttcatataacaagtatttcctaagttacgaagtccagtaagagctggtccagaacctccaaaaacaggattgaggttccgaatctgagaagcagaaagccttgagatctcagctttaggataacatgttggcttgttttcccgattaactgttggagttactgttggcttcctcttctcttcctcttgaatagcctgggttatatctggggaggagtaggagcgcttcagtttggaaggttccctatcccgctcagcaggaatctgtggcttggctttatgagttggaggggtggaaggaggtgcagatgaaggagccatttccggtgggtacatatgaacagtgttggtgggtgaatgataataacgaaaggttccagtgattgggtcaagaaacttggcccagcctgaaggcagtcctggtacgatcctccccatttcttcacttcgtgctcttgtcaaaggttctcgttgagctttatttctttcggtatcgtctgtatcctctctaaaagttcctgtccttagaattccactttctggttgtcctttaatcttaaatggcttgcctgaacctgaatcccctgtcacagatgtatggggcacatctcctgttgactttttctgtatttctggggttggacaccttttccccctatcttctacagatttcttggcatcagaagtttcatgttcacttttactttgtctttttactcctgttatttctttgcccctctttgctgaggtttctttatcttctttcttggcctgttcactttctttcttctccatttcttcttttgctttttgttgcttctctgtaatttcattttcttcagcttcttgtttctttttggctttttgttcttgttcttccttcctcagtttctctttctgttcctcttgctgcctttcccgaagttctttttcttgtttgtttttttccattagaagagcagtttctgcatgaatacgagccttttcttcatctgttaacatgagagttggagaaaaaactactggcttggtggaacgatcaggaataacttttccactctgaggagattgttgctcatggtttgtactttcagattttattctatgctcttcaggcaatttgactgctggttttttagtacgatcaatctgtggaacattctttatactaggcactggctgaattatgggtgaaacatcagatttagaagcagcaactggttcaactggagttgatatattcagtggtcccattctctcattttgaccacttatcaattctatattttcatctacttctatagatgcaggtggcgtctgggcagcaggtttagaaggaattgattcttccaatgagggataagtaaaatccaatgagatagacacctcttcattctggcgtcgtgggggtggagtgaccttagcatttgttgtatactggggataacaaaggagccagttttcatagcctccctctaaaaccaaaggctcattgcgcaggacagttttactttcccacttgaaaagtgcatctttcagactccggagagttgttccaatctgtaaatctttggcagaactaaaccagtcaagaagtaccacatactccacattccccctcttcttccatgtgtctttagaatcatctggcaggtgtgcttcaatccaactagcagtgactcctggactgatggcttcttcaggaacactgagagaatgtaaaatacaggaatcctgataatcctgcattcttcgagcatccattataatcaagctgatgtttttatccgtcatcattgtgtatagttcctttgctgtgattgctcctttctctttggtctcacatttttcattcttttcaccattgctcttttgggttttgtctttggaatccaaaacattctccaaagagcctttagccaatgtgccaccatcctctcttcctgtttcctgccttttttgttgtagccgctgtgcttcctcctgcctgtctttttcctcaagttttttccggacttcagcttcttcatatcttaatttaaggctttcagagagtctttcagcttcttcgacagcttttttgatgtttccaggtccaagtattgaatggaaataatcctgctgttgcttgaaatcaggtctttttttgataagattataaacagtcacgtatttcatatatagtacataggccctttcctcatcacgatctaatctgcattcttctgctgtcttaaagatcttcagggcactgtgcacataactcttagtgcttattttctctggtttaacttctgtcttcttattaaggtcttttagtgaagaactgaggtagagttctttaggaactgaagccacagcaggcatgatgaattatctttacttttccactttcacaatggatgctatatttccttacaagtgcttctttccgtgacgccgggcgcgcttcactaacgccagccttctcgccaaatgcccatctcccaagaactcgagggagaattagccttggctaccaggacggaagccagcccagctc

SEQ ID NO: 14258 - RNA, 9316 nt, Homo sapiens
  source 1..9316: mol_type = other RNA
gctgggattacaggcatgagccaccgcgcccagtccggtttattcattttctgtgtcctaatatcttcattaagttaatttccagtacagttgtacctcagtatctgcagggagttggttccaggatccctttgactatcaaaatccacagatgctcaagggccctatataaaatggtgtcttttctggtgttttttgtttttgttttttgagacaaggtctcattctgttgccaggctggagagcagtggctcagtcacagctcactgtagcctcgacctcctgggctcaggtgattctcccacctcaacctaccaagtagctgggactataggcacgtgccactatgcctggtcaatttttgtattttgtgtagacagggttttgccatgttgcccaggctggtctacaactcctgggctcaagcagtctgcccacctccatcccccaaaaacgttgggattacacgtgtgagccaccatgccaggcctggagtagtatttgcatgtaacctatgcacatcctcccatatactttaagtcatctctggattacttataatatctaatacaatataaatactatgtaaatagttgttacactgtattttaaaatatgtatatttttattgttgtattattttttcaaatctttcccatcacattagttgattctgaagatgcagagcccgtaaatatggacggccaactatgttgtatttctcatttctgaaaattctatttagtttctaaagtttgtttccttcttctaaatatatttaaatatactttatttgtagcctctgcttaataattctattatctaaagtccttgggggtttaaatcttattgccttctgactcttatgataaattgtttccttgcatgttctattattttgaattgtgatctcaacttcattggggtttcatatgtggatatcctgttaggtctgagttaacatgcaacaatctagaaattctgtttccttctggcaactgccctagaaatacttttcatattaagttcacaggattcgcagaccacacaggtagtataaatttgaatcccaaactggtgaaaaggtaggtctatggtgacaaattcccaggaatgacttttattctctgtaccatgagtccaagctaacacaagcactagagggtggattttgttttttaatccttccattgagggtgaatgtctttaaaggtcctggctttgtatgtggatctcaatccaacttctcaccttgtaggggggcctaagactttacctcgagtgtccttgcgtgacctttaaaacccgagcatactggttacagaaactagggactgtctttacgcccaggcagtcacaaagcataaaccacacaccatactgttgttaaatttcctgtttagggctccgcccaggctggaatgcaatggcatgatctcagctcactgcaacctccatctcccaggttcaaatgattctgcctcagcctcccaagtagctgggattaccggcatgcgccaccatgcccagctaatttttatatttttagaagagatggattttcaccatgttggccaggctagtctcaaactcctgacctcaagtgatccgcctgcctcagcctcccaaagtgctgggattacaggcgtgagccaccaggcctggcggaaccttgatcttttaaatgtgaatttcagatatttctattacctgtaaggagagaggtggggaagacgaaggttgaagggaatattgaataaataactcctgtgtactagccctcaatacatgagatatttgataacagctatacaaaacaagccatgttaatagatgagaaattaaagctcagaaaggtcaaataatttcgctaaggtcacaatgtactattacacccgaattcacgttggaattaactagtcagatccattttcattctggacatggtggtgtatgcctgtagtcccagctatttgggggcctgaagtgagaggactgcttgtgcctaggaattcatgtacagcctgggcaacatagcaagaaactgcttctaaaaataaataggctgggtgcagtggctcacgcctgtaatcccagcactttgggaggtggaggcaggtggatcacttgaggtcaggagttcaagaccagcctggccaacacggcgaaaccccatctctactaaaaatacaaaaaattagctgggtgtggtggtgcgtgcctgtaatcccagttacttgggaggctgaggcaggagaagagctttaacccaggaagcagaggttgtggtgagctgagatcacgtcactgcactccagcctgggcaacagagcaagactctgtctcaaataaaaataaataactttgggaggccgaagtgggaggatcccgaggtcgagatcgagaccatcctggctaacacagtgaaaccccatctctactaaaaatacaaaaaattagctgggcatggtggcaggcacctgtagtctcccagctacttggaaggctgaggcagaagaattgcttgaacctgggaggcggaggttgcagtgagccgagatcgtgccactgcattccagcctgggcaacagagagagactccatctcaaaaaattaaaaataagttaacaaataatcaattttcttcctctacagcagaggtcagcaaacttattctgttaaaggccaaacagtaaatattttaggcctcataagccatatggtattggctgcaactattcagttttactgttgtatcattaaagcagccactgaaaagtgtaaacaaatgagcatgactgtgttcccataaaactttaaggacattgacatttgaatttcataaaattttcacatataacaatactattattacttggatcttttccccaaccatataaaaatttaaaacccgttgctaatgcatgggtcttacaaaaacagcctggagttgacccacgggccgtggtttgctgacccttatcatacaccataacacctccttggaagtacacctctctaatgcctttgttccaaacaatactgggttaggaaagacatggaaaaaggaaaatgagatacattattttttgtaccctatgggggattgaggggttgttgctacatagccccctcaatttgtgctgtagcaatatgcagttaagatccttattctaatgttaaatgtctcttctgtggcttatcctaactttaaaaaaaaaaaaaagaagccatcttacgtaaatgaacttacaattttaagacagggtctcactctgtcacccaggctggagtgcagtggtacaatcacggctcattgcagcctcgacctctcaggctcgagagatcctcccaccccaacttcccaagtagctgggactacaggtgtgcaccactatgcctagctcatcttttttttttttttttttttcctttaaaagatatggagtctcgctattttgcccaggctggtcttgaactcctggactcaagcaatccacctgcctcagcctcccagagtgttgggattacaggtgtgagccactgtgcccggcctgaattatcttcttattgtaaaatttcctttaatgcttaatagttgatgtatattaagtgctaactaaatgttcactgataaacattaatcagatgctgctaaatattgtctttctttattcacagatgatagtcaatgggcacaacatataagtagttacaatgaaatgagaagcaatatagcagtcaggctatatgcatgatttaacaacaaaattatcacttccttttaatttagaataagggacaatttaaaaagcatctcttggccctatcatttctgttccagtagttagtgttcatatgtgaatactaagtttgacattcctttctcccatagaaccattttggtgatttggatggtggccactacactgctttctgcaagaattcagtcacccaggcctgatatagctttgataacacacgagtcagtgagattccagatacttctgttcaaaatgctatggatctcctgttctatagctgccagcccttttccataccaatacaaaagcgttaagagccaggaaaatggtgtttcctgaacactgcaaaacaagcagtcagcatctggtggtagagttttgcttggtcattaaactcttagaacttacttgcatcattaacatttttatgccttgtgggcatgttatacaacctttcatcttaagataaatctgtcgtccagaagatgggtcttggttcactaaaaaaggcagtgtgaatataatgcaatgctaatggatgcaggccttcaaaacactgcaattatatagtgagttcaggtttcaaaattcagtgtttatcagaaaatatctcataatcatatatattcaacaaattattttccaaagatactcatgaagctaaacaaaaataatttttgttcaaatggctcgatgagtttaagaatatgatttgaatatatttgatataataatttagccaagaagtggtctcttagactaattgtaaaacatgaaaagttgtcagcttcacaatttgaaccccatcctttcatcttctccctgagagcctgctaatggtggtctctttctgaagcacttttagaatcttatttttatatggagtgttttactgactatatatatagcaactgagtccctcggttaaataaattataagctcctttaaccctcttaatacatcactctgtaaagatgtagtttataatgcagttcactttgcaatcatgcctgactcccggcatttttactttaatatttagaatgaatattctcaatatgtgagaatactagtcttgaaagaatgactctgggtgttattatatagcacgtgtgtatataaaatctatggttttactgtcctatatttgataatacaatattaaagacagaacacccacagggttataaattatttttctcattaagattttaatgtagctgtaaatgaaattctcgttttaaaaaaattaaagtttccatttttttttttagaataaagatttagtgcacaaatacagcccaaagccaacagaaaaattgctttgccctgtcatttccctaagaaagcactgaagttaactcaaaataggctgaaagaaaaaaagcaatcctctgagttctaggtttcacaaaaggaccacgtgttaaactatgtacatcgatttgatgtgcaagtatgcaataaatatgtacacatacattcctatctgctttacatcattctagagtattcatagtatatcaagatgggatttagaaatgtgaaaaggccataacagtgaaaaggaaaaaaaaaagataacaatagtttttagaccagtcgaataataatgcttagctagttaattattttaactttggagcagactaaaaaagttgttttgaaataaatggtacctgtaagtgatgattactgcaatacttgttaaatgttatttgtcagcactgaccggaattatatagtgctagtaacacagctcccactgtcctagaattcctctaaatggccagctatagctaccattatcctgataagcatttcaagagttgtgttgctgagccttttaaaagataactagtttataacctatgtctccttatgtggctacatcagttactcgtggtcccaatgaagtataaaagaggatataagctgctgaagatttcacagaagaaacggagatatcagaaacttcatgatcatcaaacttaaaccaccgttgtcttgctgcatttttacaataggctgtgtagtggcctccatccagcccaccgtagtgatttgaaacagaaaacaaattatatttcttcaaattgttctttggaccaataacatactgtgacaagtcaagattttctaacgggaagtccacagatgtctgtaatttttgtttccacctgccatcgtaggaaaaacgtttcagatgcactaaaagcacaggtggtaacttccagatttctatcttttttagagaatcccgtcgagctctgcaatgactgcagtaaaatctgttgttatctgtgagtttttcttctttggaaaataatctaaggcaatcctgtaatgtacatttacttgtggatgctagtggtagagacaaatacatgaaggcctcaaatgtcctagactttttgtgacatgtgaggcactgtactgtagatttgaattgaccctgaaaaagtgcaacaataatagactcattgagctgcttgtgtttctgccaggcatgttctgcagctttaaagtcatcgagatgatcattattttcttctttatatctcttccgattatcagctttatttagatcttcatggagaccatccattaggaacagaagcaattcttgtgaatcttgctgactgtatcctgcaaactggtcattgatcttcccaatggtgattttaaagtcctttggactgatatatctatactgtcctgtccacagggctttcatgattataccaaattcttctgccacttcacctttatgccccaacaaatttgacctgttaatatcatcctgataacagtttcggttgaaataatcagccaaatgtggagcgttacataggcactgcaatattgagttcatataacaagtatttcctaagttacgaagtccagtaagagctggtccagaacctccaaaaacaggattgaggttccgaatctgagaagcagaaagccttgagatctcagctttaggataacatgttggcttgttttcccgattaactgttggagttactgttggcttcctcttctcttcctcttgaatagcctgggttatatctggggaggagtaggagcgcttcagtttggaaggttccctatcccgctcagcaggaatctgtggcttggctttatgagttggaggggtggaaggaggtgcagatgaaggagccatttccggtgggtacatatgaacagtgttggtgggtgaatgataataacgaaaggttccagtgattgggtcaagaaacttggcccagcctgaaggcagtcctggtacgatcctccccatttcttcacttcgtgctcttgtcaaaggttctcgttgagctttatttctttcggtatcgtctgtatcctctctaaaagttcctgtccttagaattccactttctggttgtcctttaatcttaaatggcttgcctgaacctgaatcccctgtcacagatgtatggggcacatctcctgttgactttttctgtatttctggggttggacaccttttccccctatcttctacagatttcttggcatcagaagtttcatgttcacttttactttgtctttttactcctgttatttctttgcccctctttgctgaggtttctttatcttctttcttggcctgttcactttctttcttctccatttcttcttttgctttttgttgcttctctgtaatttcattttcttcagcttcttgtttctttttggctttttgttcttgttcttccttcctcagtttctctttctgttcctcttgctgcctttcccgaagttctttttcttgtttgtttttttccattagaagagcagtttctgcatgaatacgagccttttcttcatctgttaacatgagagttggagaaaaaactactggcttggtggaacgatcaggaataacttttccactctgaggagattgttgctcatggtttgtactttcagattttattctatgctcttcaggcaatttgactgctggttttttagtacgatcaatctgtggaacattctttatactaggcactggctgaattatgggtgaaacatcagatttagaagcagcaactggttcaactggagttgatatattcagtggtcccattctctcattttgaccacttatcaattctatattttcatctacttctatagatgcaggtggcgtctgggcagcaggtttagaaggaattgattcttccaatgagggataagtaaaatccaatgagatagacacctcttcattctggcgtcgtgggggtggagtgaccttagcatttgttgtatactggggataacaaaggagccagttttcatagcctccctctaaaaccaaaggctcattgcgcaggacagttttactttcccacttgaaaagtgcatctttcagactccggagagttgttccaatctgtaaatctttggcagaactaaaccagtcaagaagtaccacatactccacattccccctcttcttccatgtgtctttagaatcatctggcaggtgtgcttcaatccaactagcagtgactcctggactgatggcttcttcaggaacactgagagaatgtaaaatacaggaatcctgataatcctgcattcttcgagcatccattataatcaagctgatgtttttatccgtcatcattgtgtatagttcctttgctgtgattgctcctttctctttggtctcacatttttcattcttttcaccattgctcttttgggttttgtctttggaatccaaaacattctccaaagagcctttagccaatgtgccaccatcctctcttcctgtttcctgccttttttgttgtagccgctgtgcttcctcctgcctgtctttttcctcaagttttttccggacttcagcttcttcatatcttaatttaaggctttcagagagtctttcagcttcttcgacagcttttttgatgtttccaggtccaagtattgaatggaaataatcctgctgttgcttgaaatcaggtctttttttgataagattataaacagtcacgtatttcatatatagtacataggccctttcctcatcacgatctaatctgcattcttctgctgtcttaaagatcttcagggcactgtgcacataactcttagtgcttattttctctggtttaacttctgtcttcttattaaggtcttttagtgaagaactgaggtagagttctttaggaactgaagccacagcaggcatgatgaattatctttacttttccactttcacaatggatgctatatttccttacaagtgcttctttcctttaggagttgtcccactcctctccgcggacagagcttgtctccggggtaaccagcagctggtggaaggaaaggcgttcatcgttcacagcggacgacttcccagagaacaggtgctagggcccaagacccgcactcaccgtgacgccgggcgcgcttcactaacgccagccttctcgccaaatgcccatctcccaagaactcgagggagaattagccttggctaccaggacggaagccagcccagctc

SEQ ID NO: 14259 - RNA, 1649 nt, Homo sapiens
  source 1..1649: mol_type = other RNA
gctgggattacaggcatgagccaccgcgcccatcctgtactcactttttcatactcctttgcaggttggctgtgataggtgtccctggccacgtcagtggagcacccaggcctcaagcagcatgctggggaagggaaaaccccccattctggtgatggaggtggccatgaccatgtctggttttcaaaggcagctttgtaagaacagaaaccagcagctccccaacatctggccctatctgctgtgcaaaccacagggaccaggacctttccggggtgccagtggcatcctctggaaccagcttctcagtggaatttcagatgctattcctggtcaattgcctttgctatgtgctatcctttaataaattctgtttctcctcatatccacctgagtcattctctgtaacctgcaaataagaactctgcctggtagatgaccctaggctctgccacttgtcagttgtccagagtcacacagctggtgagtgggtaagcccaactccctggactgccccacctgccccactgtctacccgaggagtcctggatgaagctggtgagtgccacgctgccaggtgtggcagccagaacagggatcttggagtgagtaggccaaagggtgagtaaactctaaatgggctgagagcaaaaagcatgtttttggggggaagagatgttctaccaagcctgactctttgggcaaggagagctaggaatggtttcagggccagggaccccagcctctggctctgagctgacagcaataaggatcccaaaaaatgagcacttagcagcaattaattgctaagatgcaaagaaaaattgttttgaatattaaaattatagctataacactattaggagcgtgattcagagtttatggaaacattatttatattgatttattcccagagccatcaagactccttgaaaataattaatgttgacatttccattgctgaagctaaatgttgatatcatataatgaaaattatatgcttgggatgggctgtgctctagaaagcattaaaacaaataccaacatctacagatccctccctacccccattactaatgacccagtaaccaatgggcagggctctgaggctcttcacctacaggcctctagcccagcatagccatcagcccatctgaggactctcagaagcaagggccagcaccccagggtaagcatggggctcatccagggccatgagccaggaggtgggccaggatctagacaggaagcccctttggccagatcctggtagtgactgagccactgaattgctgctggcctcaagaactgagggaaggagaaggacaagaggaggtgaggggagtgatttggctgtgactcactcaaaatctcatcttgaattgtaataatccccacatgtcaagggcgggaccaggtggagataattggatcatgggggcagtttcccccatgctgttcttgtgatagtgagttctcacaagatgtgatggttttataaggggcttcccccttccctcactctcattctctttcctgccgccatgtgaagaaggacgtgtttgcttccctttctgccatgtttgtaagtttcctgaggctttgccagccatgcaaaactgtgagtcaattaaacctcttttctttat

SEQ ID NO: 14260 - RNA, 2766 nt, Homo sapiens
  source 1..2766: mol_type = other RNA
gctgggattacaggcatgagccaccgcgcccgaccaaactgtttttaaatgataactgccccctttaaaatacttaagccttatgcagaaatcttatgtggcatataaagagacaaggcagagatgctgtggttgaaagtaacctcttgacccacctggacatccaatgagcatagtttgaaaaccactgaaataaggtatgctatccataataatgtatgctatccatgcctcctagcaattaaatttgtaacaacaatttcaagtttaagtaagacaaattaaacactgaatggaatgttgaaatctgaggaaagctagcattcaaatgagcagttaaattcattaaacagtttgctttaaaaaatattcattaagttaaaatgacaatgtaaggtttgcatataatcatactatttattgaagtagaaagaaactgaaaagtgtttacttcaaaacttcagtctagtaaactgaaattatgaatcataaaatgctgcttcttacttttgcttcctaaatcataatctaccccaactacattgaaattttcatgaaaaataaacatatcaataatgggatttacagaaaccaatttctttacaaagtcttgaccaactgtttacctgactatcccagtaaggagaattttccttcaaagatatttttaggaaaaacttttgtttctttgtttgcttttctttttaaaatggggaaaactgtaaaacataaaagaaatgcaatatatagtagaaattgcttattccaacttctaactgctcatatcaaacttctctttagaaaaatggaaaatgtatccagtacaattcaatcgacatacaatttatttttttagtaacagatttttcaaattgagctcttaaaaagtacagttaactacaaaagattaaatagatacttataaaatatatttaccctgaaatgcttaagaataaaagtgttgatgcccatgtcaatagtacattatacattacacacattatttaaatgtcattttctttccaataacgtagataaaaccacaatatttattgcttatatcaagtgcaggttaaaatccagatagcctccaaaaacaaatcctgtgataaaggatatctcaatgttggtcaggtgaaatactgtgtttgacatgtatgaatacagttgcaaaatttaccagtttttaacaaacatgaatgtctttattttagacagccatttacagtttggggttcagaggaacctgcagtcaagagtcctgagatgttgggcttgtgactgtaaatatcacttatctggttgatgtctattctactgcaccgtttttgggatatgaggcgtttgctgcagacaaacccctatgattaatgtagcactgtcagttactagtgcagaagcttgctgggcaaaattaattgtttatagggcattttgctgaaaaaacagtgtccagccaacaaaagcgccaaccaaaatgactgacataaaccccatcttagtgagaataggttgccaatataaccacctttttctttttcgttcattctcatttagcctctgtttcatctgctgcaccttctgagctgtggtggcctttctgtcctctcgaatacgtttccgtagagcactctcactgttctcctccattgtatcttgcattttagaggaaagtcctgtacatcggtcacctgtcagtttttcttcttctagacctattctgttcccattgtatttttcagtcattattttgtttggtgaatgatcaaaggcaggagataagtcttccttagaaagttctttccatcgtttctgtatactagaatctccctttatacattttgctccttctattatagccatgtatgagaatctcagttgatctggggtctgaataagacccattcggtattttctcatgttcagtaacacttgttttatgttaatatcatctcctttttccatcaaaacaagacaagtgtctaccagagagaaggtgccagagcgcccaatgcctgcactacagtggatcaccgcaggcccatggtcagggttcaaggagccagattctctcactttaaacaagaaattgagaaatgaagctggtgattcagggactccaaaatctggccaggtagtataatgaaagtgagatattgttctggtttcaccactattgatattttctaattgtagtagatgtactgtataatacgacttcacatcttctgacaagagcttcacactgaatcctgtttctttaaacagcatctcttggtcatctgttggccagtactgtgcacatttaaccgattctttctccacaatgcggttcagcatgacaactgctttggtcttctgctgccaaaccataagccagaaatggcagcatgtgttaggaagtggaccctgtgttaagatgtaactcctttgtgcctcttctatgtcaactaaactggcattaatataatcattctcagcattttgcagtttaacacgactgtgatcatatgggcttacatctctgtatctgtttcgatttctgttttctggaaacttggccactctatgaggatagtcatgggactcatttcgaatttccaagtacagcggctgccagcgacgctgagtatccaactcttcgaactcccgctcgatggtggtgggcatggctgcgggagcgagctggcgcgagcagagcctgcgccggcggagaggctcaggccccgcacgatccggggagagcgctggcgctgcggcgcatgc

SEQ ID NO: 14261 - RNA, 2759 nt, Homo sapiens
  source 1..2759: mol_type = other RNA
gctgggattacaggcatgagccaccgcgcccgaccaaactgtttttaaatgataactgccccctttaaaatacttaagccttatgcagaaatcttatgtggcatataaagagacaaggcagagatgctgtggttgaaagtaacctcttgacccacctggacatccaatgagcatagtttgaaaaccactgaaataaggtatgctatccataataatgtatgctatccatgcctcctagcaattaaatttgtaacaacaatttcaagtttaagtaagacaaattaaacactgaatggaatgttgaaatctgaggaaagctagcattcaaatgagcagttaaattcattaaacagtttgctttaaaaaatattcattaagttaaaatgacaatgtaaggtttgcatataatcatactatttattgaagtagaaagaaactgaaaagtgtttacttcaaaacttcagtctagtaaactgaaattatgaatcataaaatgctgcttcttacttttgcttcctaaatcataatctaccccaactacattgaaattttcatgaaaaataaacatatcaataatgggatttacagaaaccaatttctttacaaagtcttgaccaactgtttacctgactatcccagtaaggagaattttccttcaaagatatttttaggaaaaacttttgtttctttgtttgcttttctttttaaaatggggaaaactgtaaaacataaaagaaatgcaatatatagtagaaattgcttattccaacttctaactgctcatatcaaacttctctttagaaaaatggaaaatgtatccagtacaattcaatcgacatacaatttatttttttagtaacagatttttcaaattgagctcttaaaaagtacagttaactacaaaagattaaatagatacttataaaatatatttaccctgaaatgcttaagaataaaagtgttgatgcccatgtcaatagtacattatacattacacacattatttaaatgtcattttctttccaataacgtagataaaaccacaatatttattgcttatatcaagtgcaggttaaaatccagatagcctccaaaaacaaatcctgtgataaaggatatctcaatgttggtcaggtgaaatactgtgtttgacatgtatgaatacagttgcaaaatttaccagtttttaacaaacatgaatgtctttattttagacagccatttacagtttggggttcagaggaacctgcagtcaagagtcctgagatgttgggcttgtgactgtaaatatcacttatctggttgatgtctattctactgcaccgtttttgggatatgaggcgtttgctgcagacaaacccctatgattaatgtagcactgtcagttactagtgcagaagcttgctgggcaaaattaattgtttatagggcattttgctgaaaaaacagtgtccagccaacaaaagcgccaaccaaaatgactgacataaaccccatcttagtgagaataggttgccaatataaccacctttttctttttcgttcattctcatttagcctctgtttcatctgctgcaccttctgagctgtggtggcctttctgtcctctcgaatacgtttccgtagagcactctcactgttctcctccattgtatcttgcattttagaggaaagtcctgtacatcggtcacctgtcagtttttcttcttctagacctattctgttcccattgtatttttcagtcattattttgtttggtgaatgatcaaaggcaggagataagtcttccttagaaagttctttccatcgtttctgtatactagaatctccctttatacattttgctccttctattatagccatgtatgagaatctcagttgatctggggtctgaataagacccattcggtattttctcatgttcagtaacacttgttttatgttaatatcatctcctttttccatcaaaacaagacaagtgtctaccagagagaaggtgccagagcgcccaatgcctgcactacagtggatcaccgcaggcccatggtcagggttcaaggagccagattctctcactttaaacaagaaattgagaaatgaagctggtgattcagggactccaaaatctggccaggtagtataatgaaagtgagatattgttctggtttcaccactattgatattttctaattgtagtagatgtactgtataatacgacttcacatcttctgacaagagcttcacactgaatcctgtttctttaaacagcatctcttggtcatctgttggccagtactgtgcacatttaaccgattctttctccacaatgcggttcagcatgacaactgctttggtcttctgctgccaaaccataagccagaaatggcagcatgtgttaggaagtggaccctgtgttaagatgtaactcctttgtgcctcttctatgtcaactaaactggcattaatataatcattctcagcattttgcagtttaacacgactgtgatcatctatttcctgcattctgcattccatgtctccctgatccatccagttggtgcctttaccatcctttccatacatcctaaattcttgctgacatcaccttttcacgttgctctccactcaggtgtgacttccaactcctctctcacataaaccccacttctgtgccgatgcagtccatgacatatcttctctaactagacgctctgatggaatgcctccatgatgaactggtctgttccctgcattgaata

SEQ ID NO: 14262 - RNA, 1553 nt, Homo sapiens
  source 1..1553: mol_type = other RNA
gctgggattacaggcatgagccaccgcgcccggcaggagagtttctcaactgtgaacacctttgttaatgggaatgctcaaattgtgctggtacttctaacaccaacgactaaagagaaatcgattgcaagggaatctggttatggttatggttaaccaagttagagaagagctagggcagggggaatagaggtagattctcagtaggaaggaaattctctacaatggtggaaattctcattaacatgaaaatgtcttttcctagatctcttgaagcttttcagctgctgggttgagctggagaattgggccaaagtgctcttgcatcttctctgcaatcctaaacctcctttctgtagctccctttccttcttctgagatatggctcaacaaatgaacacaacatttgtgctaataaacccaattcagagtttttggaatgtcaggccattacatctgcttcactctttaattttcatggttggccaaacagacaatccaagttaaggccatttgaagacaaataaattgatccattgaatttatgtatcctggaggtgctgccagagaatgtccaggccagagagaaagcaattgttaagtgctcagtggagaaaaacaaagaatcttctgtactatgtaataatcatttcccagtgatgaagacaacggtacaatggatcctttttttttttttttaaagcagccagcagtcaatgaaataaggtgtgaaaaggagaaacttcctatattctttcatagagcttttttctctcctaacaccaggagcacacacacaaaaggatcagcttcatgaaatatataagctctttaagttcacttggagctggattttgatggccaaaattctcttttccttctgacattgacattcatcgttcatccacagcattgatctggtcaaaacgccactgctggcgggcttttccatcacacggacgcaggtacaaatctttattgttttcttgcaccacagcttccatgcatttcccagaaagaatgtggacaatcatcccattctcctggaagtcccagtgctgctggtggatggccaggccttcctccgtgcagttctgaagaatcacctgctcctgcctgacagcaaagcacaggtgctgtgggctgccaaagtgaatctccttcctgctggtgtgctgcaggtactgttgctgccggctgtcactgcaaggagccaacaccatgggacagcccaggatgtccccttctgcctggcagtctgcacagagcccaagtccagtgttgtggagctttccagagaaactgggcctgggttcagatgggtacagctcagggtagacattagccagaaaccagtggaatgtccgacaacccagtctcctttgcagctgcaagcgttccatgcagtctggcttctcagcctgaaattggtgatcagcttcccgatatgatctcaggagttgggcaagtgggctcaagcatgtgcactaagaggcaaaatggtggcgtttaactggtacatgaccttcctccgggaatgcgcaactggtaac

SEQ ID NO: 14263 - RNA, 3352 nt, Homo sapiens
  source 1..3352: mol_type = other RNA
gctgggattacaggcatgagccaccgcgcccggcaggagagtttctcaactgtgaacacctttgttaatgggaatgctcaaattgtgctggtacttctaacaccaacgactaaagagaaatcgattgcaagggaatctggttatggttatggttaaccaagttagagaagagctagggcagggggaatagaggtagattctcagtaggaaggaaattctctacaatggtggaaattctcattaacatgaaaatgtcttttcctagatctcttgaagcttttcagctgctgggttgagctggagaattgggccaaagtgctcttgcatcttctctgcaatcctaaacctcctttctgtagctccctttccttcttctgagatatggctcaacaaatgaacacaacatttgtgctaataaacccaattcagagtttttggaatgtcaggccattacatctgcttcactctttaattttcatggttggccaaacagacaatccaagttaaggccatttgaagacaaataaattgatccattgaatttatgtatcctggaggtgctgccagagaatgtccaggccagagagaaagcaattgttaagtgctcagtggagaaaaacaaagaatcttctgtactatgtaataatcatttcccagtgatgaagacaacggtacaatggatcctttttttttttttttaaagcagccagcagtcaatgaaataaggtgtgaaaaggagaaacttcctatattctttcatagagcttttttctctcctaacaccaggagcacacacacaaaaggatcagcttcatgaaatatataagctctttaagttcacttggagctggattttgatggccaaaattctcttttccttctgacattgacattcatcgttcatccacagcattgatctggtcaaaacgccactgctggcgggcttttccatcacacggacgcaggtacaaatctttattgttttcttgcaccacagcttccatgcatttcccagaaagaatgtggacaatcatcccattctcctggaagtcccagtgctgctggtggatggccaggccttcctccgtgcagttctgaagaatcacctgctcctgcctgacagcaaagcacaggtgctgtgggctgccaaagtgaatctccttcctgctggtgtgctgcaggtactgttgctgccggctgtcactgcaaggagccaacaccatgggacagcccaggatgtccccttctgcctggcagtctgcacagagcccaagtccagtgttgtggagctttccagagaaactgggcctgggttcagatgggtacagctcagggtagacattagccagaaaccagtggaatgtccgacaacccagtctcctttgcagctgcaagcgttccatgcagtctggcttctcagccttgctcaaggagaaggcctctgggctatgcttgtagaaggtttctttgaatgaccccagccaggtctcagcaatgcgaaccctgttcctcagggtggcctcctggtcgaggggggaatgggaatcctgattttggtagatgtgtcctacccgagagcagggaaggatttcaacagagccaccacagagccaggccttgaaagacagttcgaggttttcaccacctcgcagcgacataagagagtcatacgctccagtgttttggaagtaatgtctgtccatggccaccacctctccgggcaccacagggctcctgatggggcttatgggggactggagggccttcctcacatgctctggcaaaggttcccagtggaaatccagcttccagtccaacaccccacgctgcaggtcctttgaggggtaatactggaaagtcttccagtcaatcacatctatcaccggagataccactcggctcctgtcaccagctattctgctgaggaggggctccagccagcctgggtggcactcgcagtgggcatccatgaagacgagcacatccccggtggctctggtggcccccagcatccgggccctgatggcacccagcctcttgttgctcctgagtaacttcaccccctccagcctggccacatattcgctgagagcagacttgagttgtcccagacgagcctggaggaaagccgtggctaccttgctggctgaggtcgtccacgaggatgatctccttcaggaaggccctgggcactgtgtcgaggatgctgtgtacagtccgcaggagagtggaccaggcctcatcatggaaacagaggatgacgctggctgtgggcaggctgtcctgagggtgctgctgcagacacagtgggtgccgcacctcgggcagagccctctggagggggatgcgggcactgagtgcctcctggaggccacgtgggtccaggctgaacggggtcaactcctcttcttcagacacctccccgtcctcatcagccccccagtccctctttggggcttccttatcctgcctccttggctgcttgatgaggcggtagctcccacctctcctgccctggctctggttccttctggcctggggtaaggccacggccaccagcagctgatcctcccgcagtgagataaagggtggcaggccctccagagggctgtactcttcaccctcatcctcagcttccagtacccaatcctgggattccccaaagtccaggcggtacctggcttcagggctgtgcttgctggcttgggctgtgacagtctggtgcagggtgtggtggggagggtgcaacatcgccaccatcatcaggacgcatcccagcatcaggagcagcaggaggaactggagtctgcatggtctgtgcctgtatcgcttccttaggagcatgttgctagaacttgccaaatgcaacaggtcatgttcaagttagctttctcccgctccaggctccttcaagcttgcagcagaacctgggttgcttgttccacctggaagtttttctgccagtcacttaacctggtcctgacatttgccaacagcgtgtgcaagacctgcttccacttacaatcagaaaaccacaggacccaagtttcaccccaagtcctctctgagtggatttctttaattgccttctgaaagcccattcacagggacttcaaattgaattgcttccctccctttaccccggttttctccttgggaaaaaaataatgattccattctgctcaggtgtttctttccccctttgtataaataggttgctatgaggtgtctgggatgagctggtgggttctcagtcaagcagggctgacagccgtccctctttggacgcttccagtcaggtcagatcaacagatgtaaagccggcaggcagtgcctggtttcctttcacaca

SEQ ID NO: 14264 - RNA, 3285 nt, Homo sapiens
  source 1..3285: mol_type = other RNA
gctgggattacaggcatgagccaccgcgcccggcaggagagtttctcaactgtgaacacctttgttaatgggaatgctcaaattgtgctggtacttctaacaccaacgactaaagagaaatcgattgcaagggaatctggttatggttatggttaaccaagttagagaagagctagggcagggggaatagaggtagattctcagtaggaaggaaattctctacaatggtggaaattctcattaacatgaaaatgtcttttcctagatctcttgaagcttttcagctgctgggttgagctggagaattgggccaaagtgctcttgcatcttctctgcaatcctaaacctcctttctgtagctccctttccttcttctgagatatggctcaacaaatgaacacaacatttgtgctaataaacccaattcagagtttttggaatgtcaggccattacatctgcttcactctttaattttcatggttggccaaacagacaatccaagttaaggccatttgaagacaaataaattgatccattgaatttatgtatcctggaggtgctgccagagaatgtccaggccagagagaaagcaattgttaagtgctcagtggagaaaaacaaagaatcttctgtactatgtaataatcatttcccagtgatgaagacaacggtacaatggatcctttttttttttttttaaagcagccagcagtcaatgaaataaggtgtgaaaaggagaaacttcctatattctttcatagagcttttttctctcctaacaccaggagcacacacacaaaaggatcagcttcatgaaatatataagctctttaagttcacttggagctggattttgatggccaaaattctcttttccttctgacattgacattcatcgttcatccacagcattgatctggtcaaaacgccactgctggcgggcttttccatcacacggacgcaggtacaaatctttattgttttcttgcaccacagcttccatgcatttcccagaaagaatgtggacaatcatcccattctcctggaagtcccagtgctgctggtggatggccaggccttcctccgtgcagttctgaagaatcacctgctcctgcctgacagcaaagcacaggtgctgtgggctgccaaagtgaatctccttcctgctggtgtgctgcaggtactgttgctgccggctgtcactgcaaggagccaacaccatgggacagcccaggatgtccccttctgcctggcagtctgcacagagcccaagtccagtgttgtggagctttccagagaaactgggcctgggttcagatgggtacagctcagggtagacattagccagaaaccagtggaatgtccgacaacccagtctcctttgcagctgcaagcgttccatgcagtctggcttctcagccttgctcaaggagaaggcctctgggctatgcttgtagaaggtttctttgaatgaccccagccaggtctcagcaatgcgaaccctgttcctcagggtggcctcctggtcgaggggggaatgggaatcctgattttggtagatgtgtcctacccgagagcagggaaggatttcaacagagccaccacagagccaggccttgaaagacagttcgaggttttcaccacctcgcagcgacataagagagtcatacgctccagtgttttggaagtaatgtctgtccatggccaccacctctccgggcaccacagggctcctgatggggcttatgggggactggagggccttcctcacatgctctggcaaaggttcccagtggaaatccagcttccagtccaacaccccacgctgcaggtcctttgaggggtaatactggaaagtcttccagtcaatcacatctatcaccggagataccactcggctcctgtcaccagctattctgctgaggaggggctccagccagcctgggtggcactcgcagtgggcatccatgaagacgagcacatccccggtggctctggtggcccccagcatccgggccctgatggcacccagcctcttgttgctcctgagtaacttcaccccctccagcctggccacatattcgctgagagcagacttgagttgtccttgctggctgaggtcgtccacgaggatgatctccttcaggaaggccctgggcactgtgtcgaggatgctgtgtacagtccgcaggagagtggaccaggcctcatcatggaaacagaggatgacgctggctgtgggcaggctgtcctgagggtgctgctgcagacacagtgggtgccgcacctcgggcagagccctctggagggggatgcgggcactgagtgcctcctggaggccacgtgggtccaggctgaacggggtcaactcctcttcttcagacacctccccgtcctcatcagccccccagtccctctttggggcttccttatcctgcctccttggctgcttgatgaggcggtagctcccacctctcctgccctggctctggttccttctggcctggggtaaggccacggccaccagcagctgatcctcccgcagtgagataaagggtggcaggccctccagagggctgtactcttcaccctcatcctcagcttccagtacccaatcctgggattccccaaagtccaggcggtacctggcttcagggctgtgcttgctggcttgggctgtgacagtctggtgcagggtgtggtggggagggtgcaacatcgccaccatcatcaggacgcatcccagcatcaggagcagcaggaggaactggagtctgcatggtctgtgcctgtatcgcttccttaggagcatgttgctagaacttgccaaatgcaacaggtcatgttcaagttagctttctcccgctccaggctccttcaagcttgcagcagaacctgggttgcttgttccacctggaagtttttctgccagtcacttaacctggtcctgacatttgccaacagcgtgtgcaagacctgcttccacttacaatcagaaaaccacaggacccaagtttcaccccaagtcctctctgagtggatttctttaattgccttctgaaagcccattcacagggacttcaaattgaattgcttccctccctttaccccggttttctccttgggaaaaaaataatgattccattctgctcaggtgtttctttccccctttgtataaataggttgctatgaggtgtctgggatgagctggtgggttctcagtcaagcagggctgacagccgtccctctttggacgcttccagtcaggtcagatcaacagatgt

SEQ ID NO: 14265 - RNA, 11182 nt, Homo sapiens
  source 1..11182: mol_type = other RNA
gctgggattacaggcatgagccaccgcgcccggcaggagagtttctcaactgtgaacacctttgttaatgggaatgctcaaattgtgctggtacttctaacaccaacgactaaagagaaatcgattgcaagggaatctggttatggttatggttaaccaagttagagaagagctagggcagggggaatagaggtagattctcagtaggaaggaaattctctacaatggtggaaattctcattaacatgaaaatgtcttttcctagatctcttgaagcttttcagctgctgggttgagctggagaattgggccaaagtgctcttgcatcttctctgcaatcctaaacctcctttctgtagctccctttccttcttctgagatatggctcaacaaatgaacacaacatttgtgctaataaacccaattcagagtttttggaatgtcaggccattacatctgcttcactctttaattttcatggttggccaaacagacaatccaagttaaggccatttgaagacaaataaattgatccattgaatttatgtatcctggaggtgctgccagagaatgtccaggccagagagaaagcaattgttaagtgctcagtggagaaaaacaaagaatcttctgtactatgtaataatcatttcccagtgatgaagacaacggtacaatggatcctttttttttttttttaaagcagccagcagtcaatgaaataaggtgtgaaaaggagaaacttcctatattctttcatagagcttttttctctcctaacaccaggagcacacacacaaaaggatcagcttcatgaaatatataagctctttaagttcacttggagctggattttgatggccaaaattctcttttccttctgacattgacattcatcgttcatccacagcattgatctggtcaaaacgccactgctggcgggcttttccatcacacggacgcaggtacaaatctttattgttttcttgcaccacagcttccatgcatttcccagaaagaatgtggacaatcatcccattctcctggaagtcccagtgctgctggtggatggccaggccttcctccgtgcagttctgaagaatcacctgctcctgcctgacagcaaagcacaggtgctgtgggctgccaaagtgaatctccttcctgctggtgtgctgcaggtactgttgctgccggctgtcactgcaaggagccaacaccatgggacagcccaggatgtccccttctgcctggcagtctgcacagagcccaagtccagtgttgtggagctttccagagaaactgggcctgggttcagatgggtacagctcagggtagacattagccagaaaccagtggaatgtccgacaacccagtctcctttgcagctgcaagcgttccatgcagtctggcttctcagccttgctcaaggagaaggcctctgggctatgcttgtagaaggtttctttgaatgaccccagccaggtctcagcaatgcgaaccctgttcctcagggtggcctcctggtcgaggggggaatgggaatcctgattttggtagatgtgtcctacccgagagcagggaaggatttcaacagagccaccacagagccaggccttgaaagacagttcgaggttttcaccacctcgcagcgacataagagagtcatacgctccagtgttttggaagtaatgtctgtccatggccaccacctctccgggcaccacagggctcctgatggggcttatgggggactggagggccttcctcacatgctctggcaaaggttcccagtggaaatccagcttccagtccaacaccccacgctgcaggtcctttgaggggtaatactggaaagtcttccagtcaatcacatctatcaccggagataccactcggctcctgtcaccagctattctgctgaggaggggctccagccagcctgggtggcactcgcagtgggcatccatgaagacgagcacatccccggtggctctggtggcccccagcatccgggccctgatggcacccagcctcttgttgctcctgagtaacttcaccccctccagcctggccacatattcgctgagagcagacttgagttgtccttgctggctgaggtcgtccacgaggatgatctccttcaggaaggccctgggcactgtgtcgaggatgctgtgtacagtccgcaggagagtggaccaggcctcatcatggaaacagaggatgacgctggctgtgggcaggctgtcctgagggtgctgctgcagacaccttcttacttctgatagttgttcaatagctatttgttcactgaaggaagaaagacactgaacttgttctcaggaagtgtgtaagttggttgtcaagattaacaggggagtaatcccacagagccaagttcctccattgcaagaaaatcctagcttgcctgtaattggtggcacttatcttgggaacaccataccaacttctaggccaggcctgaggctgctagggctgggacacagcctggagctgaggccttagaagaatggatgaagaagcttgcagacaagagagatgggaggaaagggctggagtctgcagtggaggctgattctgccagcctgtcattctccatcagtggacagacgtcacaaggtacatgccatccccttctctttgtgcaggttctccaaactctcacagctcacttctggaggggttcaggggatccttggcttgctctgatcctggcatctacctctgaaccagagacaggcacacactgggagtcactggtctgaacactgaccggaggcctatgaagcatcttggagccatagttccacctaacagggacagcctccccaggctagcggccagagaaacctgccagatcctccatctcaagaagtgtgagctttagacatgcaaaaagtgagcagttgatagcaggtcatagagcagacagtaacccaaagacggggtggtagaagccaagacgtagctcagtgcctctccggtgtccatatgcccttgaaccatccgggacctcattaaatgtagacttaggtcaagtaggtctggggtggggcctgagattctgcatttctggtgagctcccaggtaatgctgatgctgttggttcctggaccacagttagagtagagggcagtggttgttagtgacaagacaataggaggtgagctgacagatgtacagaatacttggccaggttctagggcccctactgctgcaggatgtcaggaaggccaagtccccaaaggaactgtggatcgtgggtctccctcctgtccacctccttcaaccttgtctggacagttccctgttccttacttacttcctgtgtaaacttgcagtaactccatcaccttaagtgacttgagcatctctgttcttagtcacctaaagtggcctaagcagtggtcctcagcctggttacacattagaatcacttagagagtgagttcctgtgaatcacatttacttggtctgctttggagccttgacatgacgactcattggttctaatgtgagtgggggctgtgaaccactggcctcataatggctctcaaactttaacatgaatggaaatcacctagggatcctgttaaagtagagatttcatctagtaggtttaagtggggtctgaagggtctgcatttctgaggctgcaggtctgaggaccacactgtgagtggcactggagtaaataacatcaattcctcccaccccaggacaaggtgcagattaaccacatctaatctaacccccaaggccagctgggtttgtcctgaagtgcagggtaagaccctaccacacttgttaccatgaatgcatttgacccaaaaaagggcgctatatagtcagctctgtctacgctgcaaccccactgcggggtgatggatccagagtggaggtccagaggaggtactgcctctgctgcggccactgtggactcgagggctggaaggttggtgtttgtggcatcccttcacgacttggacagccaggccccataagcaccactcacactgcccatactgggttgtcttccctctcttgtggggggaattgagctaagttccagccccaggtctcaagcccagcttgttcctgttcttgtccctcatcccgaagggcatgtctgctctcttggatttactgatgccctgtcagctgcctccttcctcttttgcaggccaggctatcacagccaacaaggggtgtggggagtcatcttggggtgaatcacggcctggcaggacagagtcttcacagggaactgagtggaccccgcgtggattgcaacaccatcttctacttgacaacaaagctgcagccaaggcgactctcccgcccctgcccttccctctgaccccttgcccattatggcctctggggcaggaagtggggaacaaagcagaagatatccctcccagctctccccaccagctgtgaagagccattgaccacctggggccttgcagcctggcttcacgatagaaccacctggggagttttaagctcttggtgcccaggcctcaccccagaccaactaaatagaaatccttggaagtggagcatgagtatgaatagtttttaagactttccagataattccaatgtacctgcacatttatgatgatttagcagcctccagggccagaaaataacttttcagtcagaaaaaggacagcaatatgatatccacagctccatttttctccatcactccaacttactcctaggccatttactcaagaatatgataagggcaacttctgtttggacttaatacacaaggaaaatcatcacacgttgtgtctcattttctctacaaccttatgcaagggtgttattattatcccattttacagttgaggaactgaggctcagagaggttgagtgacttgtacaaggtcacacagtaacaggtggtaccaggattcaaccacaggtccacaactgtttaatcacagctatgggtacataaaccagggaaacacaggctgaaccataaaggcaagttaaaagcaggtagcacacagccagctaccgctgagttgacatttatgtttagggacaaactgccggggccatgagggagcctgttcctctctgctctcttttctattttctgactctagtattgcttcctacgtggaaacttcccaaactctaccagctctccactcgctttctctaccagtagttccccagactatctagcatcagcttaaaaaaattctgattactgggctccaactcagaactctggagcattgccagtgagggggtctgaacatctacgtctttttaacaagcaatataggggggttgggtgtgcacatacttttgggaagtcgtggtgtaactcctcactgttgaaaaatgtgctctgtgggccaacagtgctggtgccaccttggagtgcctttgatagaaatggagcatctgaggctgccctcctgacctgctgaatttgactgcattttaacaggatgcctagaagattcgcatgcaccttaaagtttgaggagcactgctctggccagtctgttcggcataaagagtgtgccttagagcagaggttctcaaagtgtctctggattgggagcagcagcagcagcagtaccaggagtttgcagaaatgcaaatgttgagccccacttcacacccactgaatcagaaactggaggaatggaggccaggaatctgtatttttaacaagccatctagttgttcggatgcacgctcaagttcagccgtagatgtagattacaaagcactggctcacacagcagcctctttgatcctaggaacccattgcccctgcactggataccaggatgatcaaaggagagctggggcctggaagaactttgaaaaccatccgtgctacaggaggctaaatgggccgggcttgttcctcccgccccttctttgacagcagctttgaagggctgagttaatcccgttcctgtttgcggttccatcatgggctcttctctattttgcctcagtattcattcagttttatccccacctctgccccgaggaccctccctttcccacagcacaaccatttcattgagtttgttctgttcctgtaaagaatggattggttagtttgcatggatttacatttcccctaatgatacagtgctgtaggccgctttctgtgccttactttttcactcagcaggggatttttagggtctcccttcattgttgaatgtacccagagtctgttgcttctaactcaggctgagtatctcatagggtgcacccagctcctcctgccctgtgacaagacatcctggtggcttccagctcctcagcaccatcaaggatgctgtgataagcatttccgcaactgtctccccatggacccgtgtgagttctccccattttaagatgaaaacacttccagcccatgtgacttgcccaatctctggtctggagagtggcagactggcaaagtgtagtgtggtggttaagagtatgactttggtgtcagactcacctggtcagataacctggcaccagtccctccatctttctgtgcctcagtttcctcatccatgaaatgaaacctaccttagaggttttctatgaagagttgaaaacaaaaaccacttagcagagcctctagcacatagtaagtgctcaataaatgttcactgtaattttgcctctcttttcagagactgtcttttgacctcttttccactgatatttttcttttttgctcttgcatcattggtaattttcctcaaatgccacctattcaaactgacctccagaaatgactctaaaggtactcagaaaaaggcctgtggcctgggcaggggggaaaggacaacaggcagagctagtttgggcatttgggtgtaggaactgggccagaggggcttgtctggcttaggagtcaaggatggaattgcaaggggatgtgtggctggcgatagcacggggtgcgctacagcccgaggcacaggctcctgatgtcctagcgctctgctggtcctggtgggaaagcagcggtgcagggcccgcatactgcaggcacttaatatatgcctgtttctcttctgtgttgtattgtggcccagatttaaaggggtaggagccgaagagtcctgtcaccctggggggagggtggagatcgtttgccttgctttgcagggactctcttgtgcatgcaggcgaggaatccagttaagggaaggcgccagagcttgaaccgcagactggagaggggagtctgcagccaaggcctgggctgcgcaggccgcacgcaccagccggggccagcagagggcgctgagcacctccgcacaaagctggcggccgttccgtgagaaccctggcaagctggggattggagaatccaatcgtctcccttcgcaggggttgaggagtttcctcccgactgcctgggaccttcagtgctaaaatctgggaagtctcaggcaagtcaagacgagttggttactctggctggaagaagcaaccactgaagtgttgcacacacacataaacgcacacgtgcacatcaaacacacacagcacaaaatgtacccacacttgcaccacgcaactcacagtgcacatcacacactcatgaacatcacactacatgcataacatacacaacatgcctgcacatatacacatgtatcactcacacctcacatgtataacatacatgcaacacacaaagaatacatacgcacacatgtaccacaaaacatgtaaaacaaacactacagcacacacaggcacagtacatgcacagtacatgtgcacatcacaccacatgcacaagatacgcaatacacacgtattacacccatgcacactacacacacagcacacacaaatacgtgcacagcacacacaccacaaaatttacctgcacttgtgccacatacaacatatccatgcactttataccacatgcataataaacacaacacacttgtacatatatgcatatcccattcacacaatgcatttatagcacaatgcaccacagaagcacatcatacacaagaaacacagttacaacacaatacctgtgcacacatgcaccacgtgaacatatgcaaaacaaatagcaaactgcaacacacacccagatgaacaatgcatgtggcatcaccccaatacacaatacatatatgaaccatgcacataatacatgcacattaacacacatgcacacaagatgacacattgcacaatgcatagctgtgcatatcatatcacatacacaaagtaacatgcaccaagcatataggcaccacataacgcagtacctgcatgtactacacatacatgcacgacatccatttaatacacataatgcaatgcacacacaacacagagaatatatacaacacacatgcacgaacatacatataccatgacccacaaatatgcatattcaccacacatttgcactatgcaaacacacagtcacacacacagaccactttggtagccacagaccctctcgtttcaggcaatattatttcttatcggcaaaaagaggatgctcactcttgctccaggccagtgaaaaatagtgtcaaaaaatttgaaaactatgtttgttcattcagcaatcacttctttactgcatgttgggctttgggatgtacaatacaaactcagtcctgaccttctaaggggctcacagcatagcagggaaagcaggcattcgactgataaatacatcaataatcatttggctttagttttgtaagtgctgtgagttaaaactccagggtgcaaggagggcacaaaactagaatggggtgggaatttcctgaaaatagcttttaaaggtaaggcttgaaaacagtgtagcgggtttgaaatggaagtagggtgcggtgagtgaggcacccggggcacacaatttaaggagatgttcactcccggctgctgaccctgcaattgcacaccctcgagtgtgagtggctgagcagccaggctgaggggaactagatcagggatccgaagagtgtgtggccctgcttccaactgctgccctgcacaaatgtttgctttccaggaaactctccaggctctgggaggagcaatggcctataggaaaagggacctaaatcaccaaactaaaactaacaagctgccttgctccctggatgctggtaaccaaggctccctcctcagtggtcagccatggtgacagtaagggagcagggggtgtggaggatgggccagcatctccctgggcacagctctgcccatcacctacacttctcagcttacctcctggggctggggctgccctggcagggtaaattgcagtcagcacagtattctggctctcaggcactggacctgtttccttagtctagtggcccaaggcaggtggcatggagtggtgggtcaggcagactggagctcacatgcctgcattcaaatcctgactttgttacctactagcagcgtgactgggaaagcaacttcaccttgttttcatacctatagaataagcatgatgatactactagcacccatcttgcagagctgtgaggactttccaggactttatgagttaatacattaaaagcttgtaaagtaaatccagacgcatgggaagagccccctaaatgtaaactgcaattgttattttgatccaaactaaaagcaaacactaacaataaccctaaaatcaaaatgtagtggagtcagagtgttagaactggcaaatgtctgctctaacctcccttctgtgttatagaaataaagccatttgacctaaagacagaagaactagaacccaggacggagaagagaatgaacaagcaagagtcctcactttctgctttctaggacaatgattctcacctgaagggcttgttcatacagaccactggaccccacccagagtttcttgtttggcaggtctgggatggggtctgagaatctgcatttctgagaacccaccagtgcccaggggctgctgacgctgctggcccaggtactgcatcttgaaaagcacttgctctaagtcaggagaggcaggctacggaaagtttgcattcccgagtttgctaccacccgatcatgccctgggatcagggaagggaaaacaagggccttacttacagtgggtgccgcacctcgggcagagccctctggagggggatgcgggcactgagtgcctcctggaggccacgtgggtccaggctgaacggggtcaactcctcttcttcagacacctccccgtcctcatcagccccccagtccctctttggggcttccttatcctgcctccttggctgcttgatgaggcggtagctcccacctctcctgccctggctctggttccttctggcctggggtaaggccacggccaccagcagctgatcctcccgcagtgagataaagggtggcaggccctccagagggctgtactcttcaccctcatcctcagcttccagtacccaatcctgggattccccaaagtccaggcggtacctggcttcagggctgtgcttgctggcttgggctgtgacagtctggtgcagggtgtggtggggagggtgcaacatcgccaccatcatcaggacgcatcccagcatcaggagcagcaggaggaactggagtctgcatggtctgtgcctgtatcgcttccttaggagcatgttgctagaacttgccaaatgcaacaggtcatgttcaagttagctttctcccgctccaggctccttcaagcttgcagcagaacctgggttgcttgttccacctggaagtttttctgccagtcacttaacctggtcctgacatttgccaacagcgtgtgcaagacctgcttccacttacaatcagaaaaccacaggacccaagtttcaccccaagtcctctctgagtggatttctttaattgccttctgaaagcccattcacagggacttcaaattgaattgcttccctccctttaccccggttttctccttgggaaaaaaataatgattccattctgctcaggtgtttctttccccctttgtataaataggttgctatgaggtgtctgggatgagctggtgggttctcagtcaagcagggctgacagccgtccctctttggacgcttccagtcaggtcagatcaacagatgtaaagccggcaggcagt

SEQ ID NO: 14266 - RNA, 876 nt, Homo sapiens
  source 1..876: mol_type = other RNA
gctgggattacaggcatgagccaccgcgcccggccaaatgaaactttcctttaaggaacaagtgcatttttaatagattctggaactcggcttgcatagtagtcataattcctcagtgtggccaggactcctgcagagttcatatgcttcacatccttgtggtactgaagaacattcccatggatatcggttaacttgcctcccacagcatgtaaaataacttctggagcacaagtatcccacttcttacaaccaggacttgcaaatacataagcagaggctttgccttcaatcagctgaataatctcatagttgtaatatggctggttaataactcctgctatggcttttccttcataagcaattccaataagaactgttacattgtcaagaagaccttcggtatattccttggttccatccagaggatcaacccagaccacgagatcttcttctttaatagcactgtactgcgatgggcatggttgcttcagtatttcttcccactgactgtcttcaatcagctcttgatccacttcctcagaaggcagatcctcttcccctataattgtgagtttggggaatttccgggccaatgaagaacatatgctcatctgtgccaatcggtcagctttggtctgcaggtctgttgcacaggtctggaacaacgttggaccaaagacacttcaggaggagcaaaagcgcgttatcgtagacccaggtccctcgttgtgtccagtaccgagctttggcactgtcaataagtcttttgagaaggatggcatccctacctcagctactgagcatgcgggaaactgcgcgcaagcgcacaacagcgatttcacactgcctctttagactcctgatccgcgggaa

SEQ ID NO: 14267 - RNA, 929 nt, Homo sapiens
  source 1..929: mol_type = other RNA
gctgggattacaggcatgagccaccgcgcccggccaaatgaaactttcctttaaggaacaagtgcatttttaatagattctggaactcggcttgcatagtagtcataattcctcagtgtggccaggactcctgcagagttcatatgcttcacatccttgtggtactgaagaacattcccatggatatcggttaacttgcctcccacagcatgtaaaataacttctggagcacaagtatcccacttcttacaaccaggacttgcaaatacataagcagaggctttgccttcaatcagctgaataatctcatagttgtaatatggctggttaataactcctgctatggcttttccttcataagcaattccaataagaactgttacattgtcaagaagaccttcggtatattccttggttccatccagaggatcaacccagaccacgagatcttcttctttaatagcactgtactgcgatgggcatggttgcttcagtatttcttcccactgactgtcttcaatcagctcttgatccacttcctcagaaggcagatcctcttcccctataattgtgagtttggggaatttccgggccaatgaagaacatatgctcatctgtgccaatcggtcagctttggtctgcaggtctgttgcacaggtcttctccacaatacccaggtctccttcagcaataacacgtctgactatcattcctgccttttgagcaatagaatatgcggaggctaccaaccgcatcaacacagtgttactggaagccatggtacactctggaacaacgttggaccaaagacacttcaggaggagcaaaagcgcgttatcgtagacccaggtccctcgttgtgtccagtaccgagctttggcactgtcaataagtcttttgagaaggatggcatccctacctcagctact

SEQ ID NO: 14268 - RNA, 1038 nt, Homo sapiens
  source 1..1038: mol_type = other RNA
gctgggattacaggcatgagccaccgcgcccggccaaatgaaactttcctttaaggaacaagtgcatttttaatagattctggaactcggcttgcatagtagtcataattcctcagtgtggccaggactcctgcagagttcatatgcttcacatccttgtggtactgaagaacattcccatggatatcggttaacttgcctcccacagcatgtaaaataacttctggagcacaagtatcccacttcttacaaccaggacttgcaaatacataagcagaggctttgccttcaatcagctgaataatctcatagttgtaatatggctggttaataactcctgctatggcttttccttcataagcaattccaataagaactgttacattgtcaagaagaccttcggtatattccttggttccatccagaggatcaacccagaccacgagatcttcttctttaatagcactgtactgcgatgggcatggttgcttcagtatttcttcccactgactgtcttcaatcagctcttgatccacttcctcagaaggcagatcctcttcccctataattgtgagtttggggaatttccgggccaatgaagaacatatgctcatctgtgccaatcggtcagctttggtctgcaggtctgttgcacaggtcttctccacaatacccaggtctccttcagcaataacacgtctgactatcattcctgccttttgagcaatagaatatgcggaggctaccaaccgcatcaacacagtgttactggaagccatggtacactctggctcttgccctgaccggccggagagaaacggtgacaaacctggaacaacgttggaccaaagacacttcaggaggagcaaaagcgcgttatcgtagacccaggtccctcgttgtgtccagtaccgagctttggcactgtcaataagtcttttgagaaggatggcatccctacctcagctactgagcatgcgggaaactgcgcgcaagcgcacaacagcgatttcacactgcctctttagactcctgatc

SEQ ID NO: 14269 - RNA, 960 nt, Homo sapiens
  source 1..960: mol_type = other RNA
gctgggattacaggcatgagccaccgcgcccggccaaatgaaactttcctttaaggaacaagtgcatttttaatagattctggaactcggcttgcatagtagtcataattcctcagtgtggccaggactcctgcagagttcatatgcttcacatccttgtggtactgaagaacattcccatggatatcggttaacttgcctcccacagcatgtaaaataacttctggagcacaagtatcccacttcttacaaccaggacttgcaaatacataagcagaggctttgccttcaatcagctgaataatcttatttcctgctcctcctactcgcagcacagcatcggggttcatagcagcaacacagtcagtaaccaacttgttgctatgggatcgagtagttgtgataatgtgtttcccagcagggacttctttcagctgaaacccaaaggcgcctaaacctaaaactccccagattgtcctccccaacacagcatctggtcctgcctcatagttgtaatatggctggttaataactcctgctatggcttttccttcataagcaattccaataagaactgttacattgtcaagaagaccttcggtatattccttggttccatccagaggatcaacccagaccacgagatcttcttctttaatagcactgtactgcgatgggcatggttgcttcagtatttcttcccactgactgtcttcaatcagctcttgatccacttcctcagaaggcagatcctcttcccctataattgtgagtttggggaatttccgggccaatgaagaacatatgctcatctgtgccaatcggtcagctttggtctgcaggtctgttgcacaggtctggaacaacgttggaccaaagacacttcaggaggagcaaaagcgcgttatcgtagacccaggtccctcgttgtgtccagtaccgagctttggcactgtcaat

SEQ ID NO: 14270 - RNA, 1002 nt, Homo sapiens
  source 1..1002: mol_type = other RNA
gctgggattacaggcatgagccaccgcgcccggccaaatgaaactttcctttaaggaacaagtgcatttttaatagattctggaactcggcttgcatagtagtcataattcctcagtgtggccaggactcctgcagagttcatatgcttcacatccttgtggtactgaagaacattcccatggatatcggttaacttgcctcccacagcatgtaaaataacttctggagcacaagtatcccacttcttacaaccaggacttgcaaatacataagcagaggctttgccttcaatcagctgaataatcttatttcctgctcctcctactcgcagcacagcatcggggttcatagcagcaacacagtcagtaaccaacttgttgctatgggatcgagtagttgtgataatgtgtttcccagcagggacttctttcagctgaaacccaaaggcgcctaaacctaaaactccccagattgtcctccccaacacagcatctggtcctgcctcatagttgtaatatggctggttaataactcctgctatggcttttccttcataagcaattccaataagaactgttacattgtcaagaagaccttcggtatattccttggttccatccagaggatcaacccagaccacgagatcttcttctttaatagcactgtactgcgatgggcatggttgcttcagtatttcttcccactgactgtcttcaatcagctcttgatccacttcctcagaaggcagatcctcttcccctataattgtgagtttggggaatttccgggccaatgaagaacatatgctcatctgtgccaatcggtcagctttggtctgcaggtctgttgcacaggtctggctcttgccctgaccggccggagagaaacggtgacaaacctggaacaacgttggaccaaagacacttcaggaggagcaaaagcgcgttatcgtagacccaggtccctcgttgtgtccagtaccgagctttggcactgtcaat

SEQ ID NO: 14271 - RNA, 1088 nt, Homo sapiens
  source 1..1088: mol_type = other RNA
gctgggattacaggcatgagccaccgcgcccggccaaatgaaactttcctttaaggaacaagtgcatttttaatagattctggaactcggcttgcatagtagtcataattcctcagtgtggccaggactcctgcagagttcatatgcttcacatccttgtggtactgaagaacattcccatggatatcggttaacttgcctcccacagcatgtaaaataacttctggagcacaagtatcccacttcttacaaccaggacttgcaaatacataagcagaggctttgccttcaatcagctgaataatcttatttcctgctcctcctactcgcagcacagcatcggggttcatagcagcaacacagtcagtaaccaacttgttgctatgggatcgagtagttgtgataatgtgtttcccagcagggacttctttcagctgaaacccaaaggcgcctaaacctaaaactccccagattgtcctccccaacacagcatctggtcctgcctcatagttgtaatatggctggttaataactcctgctatggcttttccttcataagcaattccaataagaactgttacattgtcaagaagaccttcggtatattccttggttccatccagaggatcaacccagaccacgagatcttcttctttaatagcactgtactgcgatgggcatggttgcttcagtatttcttcccactgactgtcttcaatcagctcttgatccacttcctcagaaggcagatcctcttcccctataattgtgagtttggggaatttccgggccaatgaagaacatatgctcatctgtgccaatcggtcagctttggtctgcaggtctgttgcacaggtcttctccacaatacccaggtctccttcagcaataacacgtctgactatcattcctgccttttgagcaatagaatatgcggaggctaccaaccgcatcaacacagtgttactggaagccatggtacactctggaacaacgttggaccaaagacacttcaggaggagcaaaagcgcgttatcgtagacccaggtccctcgttgtgtccagtaccgagctttggcactgtcaat

SEQ ID NO: 14272 - RNA, 1201 nt, Homo sapiens
  source 1..1201: mol_type = other RNA
gctgggattacaggcatgagccaccgcgcccggccaaatgaaactttcctttaaggaacaagtgcatttttaatagattctggaactcggcttgcatagtagtcataattcctcagtgtggccaggactcctgcagagttcatatgcttcacatccttgtggtactgaagaacattcccatggatatcggttaacttgcctcccacagcatgtaaaataacttctggagcacaagtatcccacttcttacaaccaggacttgcaaatacataagcagaggctttgccttcaatcagctgaataatcttatttcctgctcctcctactcgcagcacagcatcggggttcatagcagcaacacagtcagtaaccaacttgttgctatgggatcgagtagttgtgataatgtgtttcccagcagggacttctttcagctgaaacccaaaggcgcctaaacctaaaactccccagattgtcctccccaacacagcatctggtcctgcctcatagttgtaatatggctggttaataactcctgctatggcttttccttcataagcaattccaataagaactgttacattgtcaagaagaccttcggtatattccttggttccatccagaggatcaacccagaccacgagatcttcttctttaatagcactgtactgcgatgggcatggttgcttcagtatttcttcccactgactgtcttcaatcagctcttgatccacttcctcagaaggcagatcctcttcccctataattgtgagtttggggaatttccgggccaatgaagaacatatgctcatctgtgccaatcggtcagctttggtctgcaggtctgttgcacaggtcttctccacaatacccaggtctccttcagcaataacacgtctgactatcattcctgccttttgagcaatagaatatgcggaggctaccaaccgcatcaacacagtgttactggaagccatggtacactctggctcttgccctgaccggccggagagaaacggtgacaaacctggaacaacgttggaccaaagacacttcaggaggagcaaaagcgcgttatcgtagacccaggtccctcgttgtgtccagtaccgagctttggcactgtcaataagtcttttgagaaggatggcatccctacctcagctactgagcatgcgggaaactgcgcgcaagcgcacaa

SEQ ID NO: 14273 - RNA, 952 nt, Homo sapiens
  source 1..952: mol_type = other RNA
gctgggattacaggcatgagccaccgcgcccggccaaatgaaactttcctttaaggaacaagtgcatttttaatagattctggaactcggcttgcatagtagtcataattcctcagtgtggccaggactcctgcagagttcatatgcttcacatccttgtggtactgaagaacattcccatggatatcggttaacttgcctcccacagcatgtaaaataacttctggagcacaagtatcccacttcttacaaccaggacttgcaaatacataagcagaggctttgccttcaatcagctgaataatcttatttcctgctcctcctactcgcagcacagcatcggggttcatagcagcaacacagtcagtaaccaacttgttgctatgggatcgagtagttgtgataatgtgtttcccagcagggacttctttcagctgaaacccaaaggcgcctaaacctaaaactccccagattgtcctccccaacacagcatctggtcctgcctcatagttgtaatatggctggttaataactcctgctatggcttttccttcataagcaattccaataagaactgttacattgtcaagaagaccttcggtatattccttggttccatccagaggatcaacccagaccacgagctcttcccctataattgtgagtttggggaatttccgggccaatgaagaacatatgctcatctgtgccaatcggtcagctttggtctgcaggtctgttgcacaggtctggaacaacgttggaccaaagacacttcaggaggagcaaaagcgcgttatcgtagacccaggtccctcgttgtgtccagtaccgagctttggcactgtcaataagtcttttgagaaggatggcatccctacctcagctactgagcatgcgggaaactgcgcgcaagcgcacaacagcgatttcacactgcctctttagactc

SEQ ID NO: 14274 - RNA, 980 nt, Homo sapiens
  source 1..980: mol_type = other RNA
gctgggattacaggcatgagccaccgcgcccggccaaatgaaactttcctttaaggaacaagtgcatttttaatagattctggaactcggcttgcatagtagtcataattcctcagtgtggccaggactcctgcagagttcatatgcttcacatccttgtggtactgaagaacattcccatggatatcggttaacttgcctcccacagcatgtaaaataacttctggagcacaagtatcccacttcttacaaccaggacttgcaaatacataagcagaggctttgccttcaatcagctgaataatcttatttcctgctcctcctactcgcagcacagcatcggggttcatagcagcaacacagtcagtaaccaacttgttgctatgggatcgagtagttgtgataatgtgtttcccagcagggacttctttcagctgaaacccaaaggcgcctaaacctaaaactccccagattgtcctccccaacacagcatctggtcctgcctcatagttgtaatatggctggttaataactcctgctatggcttttccttcataagcaattccaataagaactgttacattgtcaagaagaccttcggtatattccttggttccatccagaggatcaacccagaccacgagctcttcccctataattgtgagtttggggaatttccgggccaatgaagaacatatgctcatctgtgccaatcggtcagctttggtctgcaggtctgttgcacaggtcttctccacaatacccaggtctccttcagcaataacacgtctgactatcattcctgccttttgagcaatagaatatgcggaggctaccaaccgcatcaacacagtgttactggaagccatggtacactctggaacaacgttggaccaaagacacttcaggaggagcaaaagcgcgttatcgtagacccaggtccctcgttgtgtccagtaccgagctttggcactgtcaat

SEQ ID NO: 14275 - RNA, 1117 nt, Homo sapiens
  source 1..1117: mol_type = other RNA
gctgggattacaggcatgagccaccgcgcccggccaaatgaaactttcctttaaggaacaagtgcatttttaatagattctggaactcggcttgcatagtagtcataattcctcagtgtggccaggactcctgcagagttcatatgcttcacatccttgtggtactgaagaacattcccatggatatcggttaacttgcctcccacagcatgtaaaataacttctggagcacaagtatcccacttcttacaaccaggacttgcaaatacataagcagaggctttgccttcaatcagctgaataatcttatttcctgctcctcctactcgcagcacagcatcggggttcatagcagcaacacagtcagtaaccaacttgttgctatgggatcgagtagttgtgataatgtgtttcccagcagggacttctttcagctgaaacccaaaggcgcctaaacctaaaactccccagattgtcctccccaacacagcatctggtcctgcctcatagttgtaatatggctggttaataactcctgctatggcttttccttcataagcaattccaataagaactgttacattgtcaagaagaccttcggtatattccttggttccatccagaggatcaacccagaccacgagctcttcccctataattgtgagtttggggaatttccgggccaatgaagaacatatgctcatctgtgccaatcggtcagctttggtctgcaggtctgttgcacaggtcttctccacaatacccaggtctccttcagcaataacacgtctgactatcattcctgccttttgagcaatagaatatgcggaggctaccaaccgcatcaacacagtgttactggaagccatggtacactctggctcttgccctgaccggccggagagaaacggtgacaaacctggaacaacgttggaccaaagacacttcaggaggagcaaaagcgcgttatcgtagacccaggtccctcgttgtgtccagtaccgagctttggcactgtcaataagtcttttgagaaggatggcatccctacctcagctactgagcatgcgggaaactgcgcgcaagcgcacaacagcgatttcacactgcctcttta

SEQ ID NO: 14276 - RNA, 1116 nt, Homo sapiens
  source 1..1116: mol_type = other RNA
gctgggattacaggcatgagccaccgcgcccggccaaatgaaactttcctttaaggaacaagtgcatttttaatagattctggaactcggcttgcatagtagtcataattcctcagtgtggccaggactcctgcagagttcatatgcttcacatccttgtggtactgaagaacattcccatggatatcggttaacttgcctcccacagcatgtaaaataacttctggagcacaagtatcccacttcttacaaccaggacttgcaaatacataagcagaggctttgccttcaatcagctgaataatcttatttcctgctcctcctactcgcagcacagcatcggggttcatagcagcaacacagtcagtaaccaacttgttgctatgggatcgagtagttgtgataatgtgtttcccagcagggacttctttcagctgaaacccaaaggcgcctaaacctaaaactccccagattgtcctccccaacacagcatctggtcctgcctttgcttcattcctgtgttcccttaactgctgtttttcattgttctcatagttgtaatatggctggttaataactcctgctatggcttttccttcataagcaattccaataagaactgttacattgtcaagaagaccttcggtatattccttggttccatccagaggatcaacccagaccacgagatcttcttctttaatagcactgtactgcgatgggcatggttgcttcagtatttcttcccactgactgtcttcaatcagctcttgatccacttcctcagaaggcagatcctcttcccctataattgtgagtttggggaatttccgggccaatgaagaacatatgctcatctgtgccaatcggtcagctttggtctgcaggtctgttgcacaggtctggaacaacgttggaccaaagacacttcaggaggagcaaaagcgcgttatcgtagacccaggtccctcgttgtgtccagtaccgagctttggcactgtcaataagtcttttgagaaggatggcatccctacctcagctactgagcatgcgggaaactgcgcgcaagcgcacaacagcgatttcacactgcctctttagactcctgatccgcgg

SEQ ID NO: 14277 - RNA, 1172 nt, Homo sapiens
  source 1..1172: mol_type = other RNA
gctgggattacaggcatgagccaccgcgcccggccaaatgaaactttcctttaaggaacaagtgcatttttaatagattctggaactcggcttgcatagtagtcataattcctcagtgtggccaggactcctgcagagttcatatgcttcacatccttgtggtactgaagaacattcccatggatatcggttaacttgcctcccacagcatgtaaaataacttctggagcacaagtatcccacttcttacaaccaggacttgcaaatacataagcagaggctttgccttcaatcagctgaataatcttatttcctgctcctcctactcgcagcacagcatcggggttcatagcagcaacacagtcagtaaccaacttgttgctatgggatcgagtagttgtgataatgtgtttcccagcagggacttctttcagctgaaacccaaaggcgcctaaacctaaaactccccagattgtcctccccaacacagcatctggtcctgcctttgcttcattcctgtgttcccttaactgctgtttttcattgttctcatagttgtaatatggctggttaataactcctgctatggcttttccttcataagcaattccaataagaactgttacattgtcaagaagaccttcggtatattccttggttccatccagaggatcaacccagaccacgagatcttcttctttaatagcactgtactgcgatgggcatggttgcttcagtatttcttcccactgactgtcttcaatcagctcttgatccacttcctcagaaggcagatcctcttcccctataattgtgagtttggggaatttccgggccaatgaagaacatatgctcatctgtgccaatcggtcagctttggtctgcaggtctgttgcacaggtcttctccacaatacccaggtctccttcagcaataacacgtctgactatcattcctgccttttgagcaatagaatatgcggaggctaccaaccgcatcaacacagtgttactggaagccatggtacactctggaacaacgttggaccaaagacacttcaggaggagcaaaagcgcgttatcgtagacccaggtccctcgttgtgtccagtaccgagctttggcactgtcaataagtcttttgagaaggatggcatccctacctcagctact

SEQ ID NO: 14278 - RNA, 1279 nt, Homo sapiens
  source 1..1279: mol_type = other RNA
gctgggattacaggcatgagccaccgcgcccggccaaatgaaactttcctttaaggaacaagtgcatttttaatagattctggaactcggcttgcatagtagtcataattcctcagtgtggccaggactcctgcagagttcatatgcttcacatccttgtggtactgaagaacattcccatggatatcggttaacttgcctcccacagcatgtaaaataacttctggagcacaagtatcccacttcttacaaccaggacttgcaaatacataagcagaggctttgccttcaatcagctgaataatcttatttcctgctcctcctactcgcagcacagcatcggggttcatagcagcaacacagtcagtaaccaacttgttgctatgggatcgagtagttgtgataatgtgtttcccagcagggacttctttcagctgaaacccaaaggcgcctaaacctaaaactccccagattgtcctccccaacacagcatctggtcctgcctttgcttcattcctgtgttcccttaactgctgtttttcattgttctcatagttgtaatatggctggttaataactcctgctatggcttttccttcataagcaattccaataagaactgttacattgtcaagaagaccttcggtatattccttggttccatccagaggatcaacccagaccacgagatcttcttctttaatagcactgtactgcgatgggcatggttgcttcagtatttcttcccactgactgtcttcaatcagctcttgatccacttcctcagaaggcagatcctcttcccctataattgtgagtttggggaatttccgggccaatgaagaacatatgctcatctgtgccaatcggtcagctttggtctgcaggtctgttgcacaggtcttctccacaatacccaggtctccttcagcaataacacgtctgactatcattcctgccttttgagcaatagaatatgcggaggctaccaaccgcatcaacacagtgttactggaagccatggtacactctggctcttgccctgaccggccggagagaaacggtgacaaacctggaacaacgttggaccaaagacacttcaggaggagcaaaagcgcgttatcgtagacccaggtccctcgttgtgtccagtaccgagctttggcactgtcaataagtcttttgagaaggatggcatccctacctcagctactgagcatgcgggaaactgcgcgcaagcgcacaacagcgatttcacactgcctctttagactcctga

SEQ ID NO: 14279 - RNA, 1025 nt, Homo sapiens
  source 1..1025: mol_type = other RNA
gctgggattacaggcatgagccaccgcgcccggccaaatgaaactttcctttaaggaacaagtgcatttttaatagattctggaactcggcttgcatagtagtcataattcctcagtgtggccaggactcctgcagagttcatatgcttcacatccttgtggtactgaagaacattcccatggatatcggttaacttgcctcccacagcatgtaaaataacttctggagcacaagtatcccacttcttacaaccaggacttgcaaatacataagcagaggctttgccttcaatcagctgaataatcttatttcctgctcctcctactcgcagcacagcatcggggttcatagcagcaacacagtcagtaaccaacttgttgctatgggatcgagtagttgtgataatgtgtttcccagcagggacttctttcagctgaaacccaaaggcgcctaaacctaaaactccccagattgtcctccccaacacagcatctggtcctgcctttgcttcattcctgtgttcccttaactgctgtttttcattgttctcatagttgtaatatggctggttaataactcctgctatggcttttccttcataagcaattccaataagaactgttacattgtcaagaagaccttcggtatattccttggttccatccagaggatcaacccagaccacgagctcttcccctataattgtgagtttggggaatttccgggccaatgaagaacatatgctcatctgtgccaatcggtcagctttggtctgcaggtctgttgcacaggtctggaacaacgttggaccaaagacacttcaggaggagcaaaagcgcgttatcgtagacccaggtccctcgttgtgtccagtaccgagctttggcactgtcaataagtcttttgagaaggatggcatccctacctcagctactgagcatgcgggaaactgcgcgcaagcgcacaacagcgatttcacactgcctctttagactcctgatccgcgggaaaattccacttgtcc

SEQ ID NO: 14280 - RNA, 1142 nt, Homo sapiens
  source 1..1142: mol_type = other RNA
gctgggattacaggcatgagccaccgcgcccggccaaatgaaactttcctttaaggaacaagtgcatttttaatagattctggaactcggcttgcatagtagtcataattcctcagtgtggccaggactcctgcagagttcatatgcttcacatccttgtggtactgaagaacattcccatggatatcggttaacttgcctcccacagcatgtaaaataacttctggagcacaagtatcccacttcttacaaccaggacttgcaaatacataagcagaggctttgccttcaatcagctgaataatcttatttcctgctcctcctactcgcagcacagcatcggggttcatagcagcaacacagtcagtaaccaacttgttgctatgggatcgagtagttgtgataatgtgtttcccagcagggacttctttcagctgaaacccaaaggcgcctaaacctaaaactccccagattgtcctccccaacacagcatctggtcctgcctttgcttcattcctgtgttcccttaactgctgtttttcattgttctcatagttgtaatatggctggttaataactcctgctatggcttttccttcataagcaattccaataagaactgttacattgtcaagaagaccttcggtatattccttggttccatccagaggatcaacccagaccacgagctcttcccctataattgtgagtttggggaatttccgggccaatgaagaacatatgctcatctgtgccaatcggtcagctttggtctgcaggtctgttgcacaggtcttctccacaatacccaggtctccttcagcaataacacgtctgactatcattcctgccttttgagcaatagaatatgcggaggctaccaaccgcatcaacacagtgttactggaagccatggtacactctggaacaacgttggaccaaagacacttcaggaggagcaaaagcgcgttatcgtagacccaggtccctcgttgtgtccagtaccgagctttggcactgtcaataagtcttttgagaaggatggcatccctacctcagctactgagcatgcgggaaactgcgcgcaagcgcacaacagcgatttcacactgcctctttagactcctgatccgcgggaaaat

SEQ ID NO: 14281 - RNA, 6067 nt, Homo sapiens
  source 1..6067: mol_type = other RNA
gctgggattacaggcatgagccaccgcgcccggccaagaacttccttttaagatttgccctgaagggccctagagcatttcctcttccatgcagagaatcagaaagcttggattctagctctagctcccaacaattagctgtatgtaattgatgatgggtgacttcattagtgtcaaagccaaagcatattctctgtcagcttttcaaaaaaacacgcagtaaagagagattcctaccaggaaaactttgatgggtgtttttcaagtgtcatctcacagcagaagatgccccaagtggtcaaaccttgccaacagcttcaaaaaaaggtaactaggatttaactttacggtgcattttgatgtttccctttgtgtcatatctgatgataaaagaaccttaaaaaaaaaaaaaaaaaacactatccagcttctccattctgtctcctgctttactttctcttgtttacaaaatacaaatttatagctggatttgatgctgaaaatttaatacagttacctcatgtcacagataaagaacagaaatgacttgaccaagttcacattgttgtttaacggcaggaaaagcactaaagatggatagtcctgccttcctaatttgaatgctcttattctctacaggttagggtcaagttattcagtaaaacaggctatcaggaggttaagcccaaacagtgaggaaacaaattttatgatgcttgtttgactaaatgcatgcagtttacctcaagattaagggatttaaaaaaggttagaaaacagtgtaaccctatctcctggatatatctacagacttgtatttaggaattatgccaggctgttatttctaacagagctgatgatcatagatgtggcctttaaggcaggactgggtatttggttcttaaaaatgattctgtgcctgccaatcttaggaataaataatgctttcaatgatctacattctctgtctacctaaaaagtacaaagaaaaagaatatatttaatcaaagagagatgtgtcccaggtagatggtaagcaacgggaataaagtcatgatatgcccagaataaccaatgatgaatgttattagccaggtagccaccattctagtcttagtaaaataagcatcccataaatgtttatataattttaggtgtcagaatacacatcaggacaatctggactaaggaaacctgaaatttaattctgaaattaattaagtaaccatgcctaaggtgagcttgttttcttaactgtaaaatggaagtgcaacctttaactttcctcagtggctcagatgaaatactgtgaaggtacagagtaatgctatatggcacaaagcaaaaagtgctgtgcaaaagaagacagtgtgctaaatattaggaaatttctgagttccagaaaatttggatttttaagaaactatgtcatgtcaagatgtgctttggagtaacaattttcccaatattatattaagtatatactaagtatatattagaagggattatataaaaggtgttcaaaaaacaaatatcaggaaaacactaatttaagcagaatttaacaattgtttttaacttcagaatttctcagagctttgaatattatataccatgaatctccaggaaaggacaagtgagcttatgttccccaaacttatatgaccacctaatcctttttacatggaccttctcagtggagcagtgttccatagaacacacattcttactctctatttttccaaaattcctactgtttgcttcaatacaaaatcataagacactgtggctagaaattttttttcatataaacataaacgtgtactgacacatgttggtaagcattttataggttgtctattctagctttcaaataacatgactctaaatctgtaaagaccagatcactaacatagcctctttccagaaggccataatgagtacctcctcatcagatagagaatgtaccctttaagttttgtaggagtcaagtacccctttgtcttggggacagatttctgttaagacagacagaaactcttcccttgctggtccagcagcagttttcttgttccctggaccagccagaataaaaagatgacttctgccacgcatcattttgttgtttgtctaacactgaatcccaaataaaatttcattcctgattaatagatctgaccttttaaactagacaagcagcagcaacctgagatggaattgttaagagaaaaatatggtaacattcttagctaaaatactgagagaaacggagagtttaagtctactactgtctacagtacttatgtgaatgttataaaagatctgttagaaactggtggtgatggcaacaagtcctacaccagttcttaaatcctctcttatagctagtagaaaggattacaaagtttggcaaacatcttgcatgtatcaagactgttcacaggtgtctgagcaatgaataatatgtctatagattagatttaaaagctcattttacaactgtttactagatgatataaacatttttcctctcccttttgtaagctgtaggtatgcatcatagcttctgtgatctcagaaccgtttctctgaccagcaaaagaagagatgaaaatgctcctcttgacctctatctgcactacaccagaaacgtcattgagccagtttcttctaaggagataacagaaactttctatgcaaggctgtggggggctggtaatataaggctaggaggataaagctccttactaataaacaagctgacattgaataacatggcatctatgtggaacatggtttgaaaacattttaagaccattcatagacatctgagaccactcatagtttcttcctcccaaggctgtgaaataaaattcaaaagtacatcaacaaattcctggtgcttttccatcttatggtagcttacattttataccctcagtgtccttcaaaagtggctggaatagcccacctatacctttatctgatatgttcatctctttttcaccctttggagaaataagattacttataagaaaactgattctccaaaaagtatatataagtagtaagtaacactggtaaataatgggcgtttctaacagttcttagaaactggtaaggagacagaagcccataattacccccaaattcacccaccttcatacatattcacagagacatcaacagtgaatttatacataaagaataagtgaggcaaaggcaaaagcagtatcaatctgtctgagtgtaggcaatggtgctttgattatttacccgtacaaactcttcagtcccttttggttatccccaactcagctcttaagccgtagatttttgctgtggagaactcagatgtgatgtagctgctccagtaactcttttcacagtactgcatgtcaataatgggaatgatttctaatcaatttaaactgcacacggtactttaatagaacaagaagtttattactcccactcagtagttcctgggggctttgatgttaagtcatacataattcgagaaataccaggaatcttcttaatctcagtgaccatctttaataccacctctacagggatctcattgccaggtgttgcaggtataccagtcatgaagtcactagtaataaaggttcgaataaccacagatctctggcatgaaggctgcttttgaagtgggtcccgatcaaaatgtaatggtgtcaaaatcaccggcatctggctgattttcccagcatacccagactccctgagaatgttatgggcctcaaaatcagcttggcgtaaagtactgagcacccctgttgtcaagaaagtgggagtaacatctgtaggaggttctttaactggtgggccaaatatataaacaactctgttaacgttgtgacacatgcgaggtataagcctagccagaaaaataagtgattcccagtcaggttcatctttactggagattccacacacgtaactgtaggaacgacagtcaccctgcacacctacagttttaattggcagcaagaaggcattcagtgaatgcagactggtaatttgcatcagcttctcctgatcctcttctgttgtgcaggctttgactctctgtaatagggtatgtggctttttaacacttgcagaaaaatcagctactattttcaaaatattgttggtttcaggaaagtccttacaaatataaggttcttcagcacatattactctgattgccaggccaggacctggaaatggatgcctggaaactaactcttctggaagtccaagttctctgcccaaaattctcacttcatctttatgaaaatctttcagaggttctattacttttccctcctctctcaactttctgatgagctctgtgtcattgtgatgggttttgatgagttcagctttgccacttgcaacaagggatgcactttcaattagatcaggccgtaaagtaccttgggcaaggaaaacctcctctggtttcaagttcatttctccaattacttcattggcaatcttaacaaaagtatccccaatgatttttcttttctcttcaggacttgtggtcatatttaacgttttgctaattcttttccgtggggttctatcttcatctgatattggtagggttgttgttccattgtagaaagaatgagcagcatttatcactttgacctgaattccaagctttttgagggcctcttcaacagactggctttctcgttttctcataaagccattatcaatgtgcacagcaatgacttgttcttggttcaaagcacgatttagcaaagctgtacaaactgttgagtctactccaccactgagtaaaaccaaaacttttgacgtgcctactctctctttgatctctcgaatacactcaagttctctgttctgcacggtgaaggttccactgcatccagctatatcataaaggaaattcttcagtattacttttccattttctgtaaggccaacttcagggtggaactgtgctccatataactttttagattcatttgctatgcctgctactatgtttccagaacgtgccacaaccttgaatccatcagctactttgtctacactatctccatgtgtaagcaaaacaacttcttccttctgaaggcccctgaataatgaacatgtattatccacactaatgttgaaaactccatcttctctgacactttttttgtgcacagtacctccaaataccttattcatcatctgcataccatagcaaattccaagaacaggcttgccaatagtgaatattgctggatcaaaccagggagcatcttcagcatacacagaattaggtcctccagagatgataatagcacggaatccttgttcctttatagcaaatgctggtgtttccaaggggaaaatttcagactgcacgaacagttccctcactcttcggtctatgactttcccgtactgagcaccagcatccagaatgacaacagctccttcatagtggtggtggccatccttaaggtctcctccagcattctccagcaacatcagtgaggaaactggttgtgatggaaagaatggcaacgtcccaaaggaagtgactccaggaaaatacttcacattaaagcaactctttttatagtcttttatggcattgaccttttttaaagatcagaccagctttttgtagaatgtcccacactggatctctttgttgtatcatgatcagattcttggagtctccgttgcacagagccatcggggccagggccggagccgcggcggtgacggcgacagtacgagacggggcgggagggtgccggaagggtcggcgccgcgggctgaggttgagaaggaggcctggtcgaggagcagccggcagcggagaggagccagccgccagaaaagcgccgaatggagcaacagcagcggagcgcgggccccagcgccgcgggagagaagaccagcagcgcgcacgctgcccccgcctcctgcttccgccccggccggccactgggaggagccagagcccgttcggcttggcagccgagcctcagataccctccgcagccgccgccaaaccggccgg

SEQ ID NO: 14282 - RNA, 5768 nt, Homo sapiens
  source 1..5768: mol_type = other RNA
gctgggattacaggcatgagccaccgcgcccggccaagaacttccttttaagatttgccctgaagggccctagagcatttcctcttccatgcagagaatcagaaagcttggattctagctctagctcccaacaattagctgtatgtaattgatgatgggtgacttcattagtgtcaaagccaaagcatattctctgtcagcttttcaaaaaaacacgcagtaaagagagattcctaccaggaaaactttgatgggtgtttttcaagtgtcatctcacagcagaagatgccccaagtggtcaaaccttgccaacagcttcaaaaaaaggtaactaggatttaactttacggtgcattttgatgtttccctttgtgtcatatctgatgataaaagaaccttaaaaaaaaaaaaaaaaaacactatccagcttctccattctgtctcctgctttactttctcttgtttacaaaatacaaatttatagctggatttgatgctgaaaatttaatacagttacctcatgtcacagataaagaacagaaatgacttgaccaagttcacattgttgtttaacggcaggaaaagcactaaagatggatagtcctgccttcctaatttgaatgctcttattctctacaggttagggtcaagttattcagtaaaacaggctatcaggaggttaagcccaaacagtgaggaaacaaattttatgatgcttgtttgactaaatgcatgcagtttacctcaagattaagggatttaaaaaaggttagaaaacagtgtaaccctatctcctggatatatctacagacttgtatttaggaattatgccaggctgttatttctaacagagctgatgatcatagatgtggcctttaaggcaggactgggtatttggttcttaaaaatgattctgtgcctgccaatcttaggaataaataatgctttcaatgatctacattctctgtctacctaaaaagtacaaagaaaaagaatatatttaatcaaagagagatgtgtcccaggtagatggtaagcaacgggaataaagtcatgatatgcccagaataaccaatgatgaatgttattagccaggtagccaccattctagtcttagtaaaataagcatcccataaatgtttatataattttaggtgtcagaatacacatcaggacaatctggactaaggaaacctgaaatttaattctgaaattaattaagtaaccatgcctaaggtgagcttgttttcttaactgtaaaatggaagtgcaacctttaactttcctcagtggctcagatgaaatactgtgaaggtacagagtaatgctatatggcacaaagcaaaaagtgctgtgcaaaagaagacagtgtgctaaatattaggaaatttctgagttccagaaaatttggatttttaagaaactatgtcatgtcaagatgtgctttggagtaacaattttcccaatattatattaagtatatactaagtatatattagaagggattatataaaaggtgttcaaaaaacaaatatcaggaaaacactaatttaagcagaatttaacaattgtttttaacttcagaatttctcagagctttgaatattatataccatgaatctccaggaaaggacaagtgagcttatgttccccaaacttatatgaccacctaatcctttttacatggaccttctcagtggagcagtgttccatagaacacacattcttactctctatttttccaaaattcctactgtttgcttcaatacaaaatcataagacactgtggctagaaattttttttcatataaacataaacgtgtactgacacatgttggtaagcattttataggttgtctattctagctttcaaataacatgactctaaatctgtaaagaccagatcactaacatagcctctttccagaaggccataatgagtacctcctcatcagatagagaatgtaccctttaagttttgtaggagtcaagtacccctttgtcttggggacagatttctgttaagacagacagaaactcttcccttgctggtccagcagcagttttcttgttccctggaccagccagaataaaaagatgacttctgccacgcatcattttgttgtttgtctaacactgaatcccaaataaaatttcattcctgattaatagatctgaccttttaaactagacaagcagcagcaacctgagatggaattgttaagagaaaaatatggtaacattcttagctaaaatactgagagaaacggagagtttaagtctactactgtctacagtacttatgtgaatgttataaaagatctgttagaaactggtggtgatggcaacaagtcctacaccagttcttaaatcctctcttatagctagtagaaaggattacaaagtttggcaaacatcttgcatgtatcaagactgttcacaggtgtctgagcaatgaataatatgtctatagattagatttaaaagctcattttacaactgtttactagatgatataaacatttttcctctcccttttgtaagctgtaggtatgcatcatagcttctgtgatctcagaaccgtttctctgaccagcaaaagaagagatgaaaatgctcctcttgacctctatctgcactacaccagaaacgtcattgagccagtttcttctaaggagataacagaaactttctatgcaaggctgtggggggctggtaatataaggctaggaggataaagctccttactaataaacaagctgacattgaataacatggcatctatgtggaacatggtttgaaaacattttaagaccattcatagacatctgagaccactcatagtttcttcctcccaaggctgtgaaataaaattcaaaagtacatcaacaaattcctggtgcttttccatcttatggtagcttacattttataccctcagtgtccttcaaaagtggctggaatagcccacctatacctttatctgatatgttcatctctttttcaccctttggagaaataagattacttataagaaaactgattctccaaaaagtatatataagtagtaagtaacactggtaaataatgggcgtttctaacagttcttagaaactggtaaggagacagaagcccataattacccccaaattcacccaccttcatacatattcacagagacatcaacagtgaatttatacataaagaataagtgaggcaaaggcaaaagcagtatcaatctgtctgagtgtaggcaatggtgctttgattatttacccgtacaaactcttcagtcccttttggttatccccaactcagctcttaagccgtagatttttgctgtggagaactcagatgtgatgtagctgctccagtaactcttttcacagtactgcatgtcaataatgggaatgatttctaatcaatttaaactgcacacggtactttaatagaacaagaagtttattactcccactcagtagttcctgggggctttgatgttaagtcatacataattcgagaaataccaggaatcttcttaatctcagtgaccatctttaataccacctctacagggatctcattgccaggtgttgcaggtataccagtcatgaagtcactagtaataaaggttcgaataaccacagatctctggcatgaaggctgcttttgaagtgggtcccgatcaaaatgtaatggtgtcaaaatcaccggcatctggctgattttcccagcatacccagactccctgagaatgttatgggcctcaaaatcagcttggcgtaaagtactgagcacccctgttgtcaagaaagtgggagtaacatctgtaggaggttctttaactggtgggccaaatatataaacaactctgttaacgttgtgacacatgcgaggtataagcctagccagaaaaataagtgattcccagtcaggttcatctttactggagattccacacacgtaactgtaggaacgacagtcaccctgcacacctacagttttaattggcagcaagaaggcattcagtgaatgcagactggtaatttgcatcagcttctcctgatcctcttctgttgtgcaggctttgactctctgtaatagggtatgtggctttttaacacttgcagaaaaatcagctactattttcaaaatattgttggtttcaggaaagtccttacaaatataaggttcttcagcacatattactctgattgccaggccaggacctggaaatggatgcctggaaactaactcttctggaagtccaagttctctgcccaaaattctcacttcatctttatgaaaatctttcagaggttctattacttttccctcctctctcaactttctgatgagctctgtgtcattgtgatgggttttgatgagttcagctttgccacttgcaacaagggatgcactttcaattagatcaggccgtaaagtaccttgggcaaggaaaacctcctctggtttcaagttcatttctccaattacttcattggcaatcttaacaaaagtatccccaatgatttttcttttctcttcaggacttgtggtcatatttaacgttttgctaattcttttccgtggggttctatcttcatctgatattggtagggttgttgttccattgtagaaagaatgagcagcatttatcactttgacctgaattccaagctttttgagggcctcttcaacagactggctttctcgttttctcataaagccattatcaatgtgcacagcaatgacttgttcttggttcaaagcacgatttagcaaagctgtacaaactgttgagtctactccaccactgagtaaaaccaaaacttttgacgtgcctactctctctttgatctctcgaatacactcaagttctctgttctgcacggtgaaggttccactgcatccagctatatcataaaggaaattcttcagtattacttttccattttctgtaaggccaacttcagggtggaactgtgctccatataactttttagattcatttgctatgcctgctactatgtttccagaacgtgccacaaccttgaatccatcagctactttgtctacactatctccatgtgtaagcaaaacaacttcttccttctgaaggcccctgaataatgaacatgtattatccacactaatgttgaaaactccatcttctctgacactttttttgtgcacagtacctccaaataccttattcatcatctgcataccatagcaaattccaagaacaggcttgccaatagtgaatattgctggatcaaaccagggagcatcttcagcatacacagaattaggtcctccagagatgataatagcacggaatccttgttcctttatagcaaatgctggtgtttccaaggggaaaatttcagactgcacgaacagttccctcactcttcggtctatgactttcccgtactgagcaccagcatccagaatgacaacagctccttcatagtggtggtggccatccttaaggtctcctccagcattctccagcttggagtctccgttgcacagagccatcggggccagggccggagccgcggcggtgacggcgacagtacgagacggggcgggagggtgccggaagggtcggcgccgcgggctgaggttgagaaggaggcctggtcgaggagcagccggcagcggagaggagccagccgccagaaaagcgccgaatggagcaacagcagcggagcgcgggccccagcgccgcgggagagaagaccagcagcgcgcacgct

SEQ ID NO: 14283 - RNA, 5580 nt, Homo sapiens
  source 1..5580: mol_type = other RNA
gctgggattacaggcatgagccaccgcgcccggccaagaacttccttttaagatttgccctgaagggccctagagcatttcctcttccatgcagagaatcagaaagcttggattctagctctagctcccaacaattagctgtatgtaattgatgatgggtgacttcattagtgtcaaagccaaagcatattctctgtcagcttttcaaaaaaacacgcagtaaagagagattcctaccaggaaaactttgatgggtgtttttcaagtgtcatctcacagcagaagatgccccaagtggtcaaaccttgccaacagcttcaaaaaaaggtaactaggatttaactttacggtgcattttgatgtttccctttgtgtcatatctgatgataaaagaaccttaaaaaaaaaaaaaaaaaacactatccagcttctccattctgtctcctgctttactttctcttgtttacaaaatacaaatttatagctggatttgatgctgaaaatttaatacagttacctcatgtcacagataaagaacagaaatgacttgaccaagttcacattgttgtttaacggcaggaaaagcactaaagatggatagtcctgccttcctaatttgaatgctcttattctctacaggttagggtcaagttattcagtaaaacaggctatcaggaggttaagcccaaacagtgaggaaacaaattttatgatgcttgtttgactaaatgcatgcagtttacctcaagattaagggatttaaaaaaggttagaaaacagtgtaaccctatctcctggatatatctacagacttgtatttaggaattatgccaggctgttatttctaacagagctgatgatcatagatgtggcctttaaggcaggactgggtatttggttcttaaaaatgattctgtgcctgccaatcttaggaataaataatgctttcaatgatctacattctctgtctacctaaaaagtacaaagaaaaagaatatatttaatcaaagagagatgtgtcccaggtagatggtaagcaacgggaataaagtcatgatatgcccagaataaccaatgatgaatgttattagccaggtagccaccattctagtcttagtaaaataagcatcccataaatgtttatataattttaggtgtcagaatacacatcaggacaatctggactaaggaaacctgaaatttaattctgaaattaattaagtaaccatgcctaaggtgagcttgttttcttaactgtaaaatggaagtgcaacctttaactttcctcagtggctcagatgaaatactgtgaaggtacagagtaatgctatatggcacaaagcaaaaagtgctgtgcaaaagaagacagtgtgctaaatattaggaaatttctgagttccagaaaatttggatttttaagaaactatgtcatgtcaagatgtgctttggagtaacaattttcccaatattatattaagtatatactaagtatatattagaagggattatataaaaggtgttcaaaaaacaaatatcaggaaaacactaatttaagcagaatttaacaattgtttttaacttcagaatttctcagagctttgaatattatataccatgaatctccaggaaaggacaagtgagcttatgttccccaaacttatatgaccacctaatcctttttacatggaccttctcagtggagcagtgttccatagaacacacattcttactctctatttttccaaaattcctactgtttgcttcaatacaaaatcataagacactgtggctagaaattttttttcatataaacataaacgtgtactgacacatgttggtaagcattttataggttgtctattctagctttcaaataacatgactctaaatctgtaaagaccagatcactaacatagcctctttccagaaggccataatgagtacctcctcatcagatagagaatgtaccctttaagttttgtaggagtcaagtacccctttgtcttggggacagatttctgttaagacagacagaaactcttcccttgctggtccagcagcagttttcttgttccctggaccagccagaataaaaagatgacttctgccacgcatcattttgttgtttgtctaacactgaatcccaaataaaatttcattcctgattaatagatctgaccttttaaactagacaagcagcagcaacctgagatggaattgttaagagaaaaatatggtaacattcttagctaaaatactgagagaaacggagagtttaagtctactactgtctacagtacttatgtgaatgttataaaagatctgttagaaactggtggtgatggcaacaagtcctacaccagttcttaaatcctctcttatagctagtagaaaggattacaaagtttggcaaacatcttgcatgtatcaagactgttcacaggtgtctgagcaatgaataatatgtctatagattagatttaaaagctcattttacaactgtttactagatgatataaacatttttcctctcccttttgtaagctgtaggtatgcatcatagcttctgtgatctcagaaccgtttctctgaccagcaaaagaagagatgaaaatgctcctcttgacctctatctgcactacaccagaaacgtcattgagccagtttcttctaaggagataacagaaactttctatgcaaggctgtggggggctggtaatataaggctaggaggataaagctccttactaataaacaagctgacattgaataacatggcatctatgtggaacatggtttgaaaacattttaagaccattcatagacatctgagaccactcatagtttcttcctcccaaggctgtgaaataaaattcaaaagtacatcaacaaattcctggtgcttttccatcttatggtagcttacattttataccctcagtgtccttcaaaagtggctggaatagcccacctatacctttatctgatatgttcatctctttttcaccctttggagaaataagattacttataagaaaactgattctccaaaaagtatatataagtagtaagtaacactggtaaataatgggcgtttctaacagttcttagaaactggtaaggagacagaagcccataattacccccaaattcacccaccttcatacatattcacagagacatcaacagtgaatttatacataaagaataagtgaggcaaaggcaaaagcagtatcaatctgtctgagtgtaggcaatggtgctttgattatttacccgtacaaactcttcagtcccttttggttatccccaactcagctcttaagccgtagatttttgctgtggagaactcagatgtgatgtagctgctccagtaactcttttcacagtactgcatgtcaataatgggaatgatttctaatcaatttaaactgcacacggtactttaatagaacaagaagtttattactcccactcagtagttcctgggggctttgatgttaagtcatacataattcgagaaataccaggaatcttcttaatctcagtgaccatctttaataccacctctacagggatctcattgccaggtgttgcaggtataccagtcatgaagtcactagtaataaaggttcgaataaccacagatctctggcatgaaggctgcttttgaagtgggtcccgatcaaaatgtaatggtgtcaaaatcaccggcatctggctgattttcccagcatacccagactccctgagaatgttatgggcctcaaaatcagcttggcgtaaagtactgagcacccctgttgtcaagaaagtgggagtaacatctgtaggaggttctttaactggtgggccaaatatataaacaactctgttaacgttgtgacacatgcgaggtataagcctagccagaaaaataagtgattcccagtcaggttcatctttactggagattccacacacgtaactgtaggaacgacagtcaccctgcacacctacagttttaattggcagcaagaaggcattcagtgaatgcagactggtaatttgcatcagcttctcctgatcctcttctgttgtgcaggctttgactctctgtaatagggtatgtggctttttaacacttgcagaaaaatcagctactattttcaaaatattgttggtttcaggaaagtccttacaaatataaggttcttcagcacatattactctgattgccaggccaggacctggaaatggatgcctggaaactaactcttctggaagtccaagttctctgcccaaaattctcacttcatctttatgaaaatctttcagaggttctattacttttccctcctctctcaactttctgatgagctctgtgtcattgtgatgggttttgatgagttcagctttgccacttgcaacaagggatgcactttcaattagatcaggccgtaaagtaccttgggcaaggaaaacctcctctggtttcaagttcatttctccaattacttcattggcaatcttaacaaaagtatccccaatgatttttcttttctcttcaggacttgtggtcatatttaacgttttgctaattcttttccgtggggttctatcttcatctgatattggtagggttgttgttccattgtagaaagaatgagcagcatttatcactttgacctgaattccaagctttttgagggcctcttcaacagactggctttctcgttttctcataaagccattatcaatgtgcacagcaatgacttgttcttggttcaaagcacgatttagcaaagctgtacaaactgttgagtctactccaccactgagtaaaaccaaaacttttgacgtgcctactctctctttgatctctcgaatacactcaagttctctgttctgcacggtgaaggttccactgcatccagctatatcataaaggaaattcttcagtattacttttccattttctgtaaggccaacttcagggtggaactgtgctccatataactttttagattcatttgctatgcctgctactatgtttccagaacgtgccacaaccttgaatccatcagctactttgtctacactatctccatgtgtaagcaaaacaacttcttccttctgaaggcccctgaataatgaacatgtattatccacactaatgttgaaaactccatcttctctgacactttttttgtgcacagtacctccaaataccttattcatcatctgcataccatagcaaattccaagaacaggcttgccaatagtgaatattgctggatcaaaccagggagcatcttcagcatacacagaattaggtcctccagagatgataatagcacggaatccttgttcctttatagcaaatgctggtgtttccaaggggaaaatttcagactgcacgaacagttccctcactcttcggtctatgactttcccgtactgagcaccagcatccagaatgacaacagctccttcatagtggtggtggccatccttaaggtctcctccagcattctccagctttttttgaacggaaaattgaatatttgaactctccaaagccatggatactggcttctc

SEQ ID NO: 14284 - RNA, 683 nt, Homo sapiens
  source 1..683: mol_type = other RNA
gctgggattacaggcatgagccaccgcgcccggccaagacactttcaagtgttgtctccgttgccttcacacaaaccccaggagggagacagcccccgtttacagaggagcagcctgaagcctagtcttcatcaatttgaccatcataaagctcacaagtcgcaaagctgggatgaaaatccaggtcttctgactttcactctgccgcaccgaattctttgagccagcctcagcctctcatgagaaggtcactctgaatttcttgtcccatgctttgtcctggcccctctcactgagcacgccagtcccagcaccccagtcccagctaagacagtgctcttggggaggggttagcacaggccctccaatgcccagccagtcccagaccatgttcacttcctcaaagggcactcatgtctgggccatgctaaaaggtcctgggttcgtgcccaggaagagcacttccttggggccctggcagcagcgagtcacaaagttacgatgtggctcttatacaatactccacgggattgtgaatgatgcgtgcagactccaaaaactgcagttggttcagctcagcattgagccaaactcctcctccaggaagccctcagccaagccttgagggcagggcgggggctctctctgggcacctgctggctcatgcagggtccctagtgaaa

SEQ ID NO: 14285 - RNA, 3338 nt, Homo sapiens
  source 1..3338: mol_type = other RNA
gctgggattacaggcatgagccaccgcgcccggccaccctggtacctttacactctagcttgtggctactttcccggcctcatctcccagccccaccttgtacatcagcatcccagaactgttagcactgaccccaatacatcatgctcgttcacttcctcccgttttcacccaagttgttctttggccccacaagcctttctcatgcctttcatcaaccagaagatgcccactcatttcttcaagacccagaatgggcatcatattctccaggaagcctaccccaagtgctgctcactcctggcagttggtcactctgtccaccgtgtgccacggtacccacggtggtccgggttccagcaccgattgccctgcctggatggcggtgtttgatgacaataaactgcttgagagcagggctagagtctgtttcacccctggggatctggatcctaacacacttcctggtaccttagcagatggccaaaaatggcaatgggtgagtggctgaatgaacgagtgacagacacatgagtctctaagccccacggctttctcctgcacaccagacaccatgactatgcttcagcatctgtgtaattacgtgcttcctcccacaagagtgtgagctccaagggcccgtgcccatgtttgatgctgtatttcagcacatctctgcctcctactcttgcctccgagttcctgtcttccctttgtacaccattcacgttagcgtcctgcttaaacccgttccacggccctcaccactcctagaataaaatctgaactcctgacctacgagcccctgcacaatctggccctgtctgtgtctccggcctcaccttgatccccgctcacctgcctcactacccttcagccctcgctgcaagctccttcctgccccggggcctttgcacgtgctgctctgcctgccacactcctgccccagctccgccctgctggcttcttctcatcctttcactgtccactgaaatctcttcctcacaactgggttaggctcccctgatggagcatttcatagcatctcgtttctcctatagcctaactgtaatttattgtgtatgtacatgatcgattaatgcctgtctcatgcacaagatgtttactctatgagacgtcggggcccctggctgttttcctgcctcctgcacgctgagcacggagcacaatgcctagctttttaaggcgcacaaataaattgccggtaatgaatgaatgaatgagaaggccctttctgtgcctcgttcgtgtcccctgctccaatgccttcttatgtaccagtgcctggtacacagtaggtgcttaataagcccttgtggaataatgaatgaaaaaaatgaatgaatgcccgcgtccaacccttctttctgcctttctgcatcccttcgctgtgtctctttatatagggcatatatatagtttgtgggtgtaactatgtattcgtgtattatgggcccctctccaggagttgggctgggctgggagtccctccctcccctccccccgccccgccccccatgcacacagcaaaacatgaaaaagaaaacatctcgaaactgcaaaaaacaccatggccctcccccctccccatagatcccccaaaaaaataaaacacgacgctccctcacagcggccccctccctcccctgccccctccctcggggtccctgcttcggagggggaggggggcggggagggtgggcgtggggcgggcccagcagtctccagcgcgctcacgggggaaagcgggggcgcccccgaccccggcagcctcgatgcacgcgcgcccgcgcacgcgccccggacacgcccctcggctcccccgccgcgcccctacacaggcgtggttttcctgttgagcgtgttggtgttggaggcggcggcctccttggccagggtcccgggggcgggcgcagagggcgcgggtggcgcgggcgcgggcggggcgggcggcccggtgaccgtgaccgtgacgccgccgcccgcctccttggggaaggcgttgtgcagcgtgaggaagccggacgcccccccgcggtcccgctcggcacccgccccgccgccgcctccgccgccgcccccggcgcccccggccgcgccgccgaacgcccccacggcgccgccgccgccgccgccggcccccgccagccccgcggccacgctgcccttggaggggtcgcggctgagcgtgtacatggagatgtccgtggaggcaaagcccgggcccccggggccgccgggagacgcgtcccgcgacggcgacggctcgctggagcgggagctagagcgggagcggcggcggtagcggaagcggtaactgggcagacggaggatggccgaggggccgctcccgccactgccgcccgcgcccccgccggccttgagcaggtccgagcgagactggcagtgcgcctcgcggctgcgctcgatgtagatgttgacggccagcacgcctatcacctcggccaggatgaacgacagcccgccgaagtagaaggaccagccgtacgagtagtggtttttcttctcctcgtcccgcttcgggcccggctcgcccgcgttggcggagatgtacacgatcacgccgatgatgttgctcaggcctgctgccacgaacaggatccctgcgcccagaatgatgttcctcttggacttgtagacgcgggaggccgccacgcacacacccccgagcagcagcaggatggcgctaaggatggggaagatgctggaggcccggacaactcggagtagatactccgcgctgtcgtggtcgtagtccgtgtcctccgggaaatgattgatcttcacgcagacgcctcttttcaacccttccaggcagcagatcctccagaggcccgagtgcgtgaggccgccggggtccttcttctccgaggcgccgccgcccccgcggtggggggtcccgtcgtcgccgccggccgtgaggttggtggtgttgcagatgagggcgcgcgtgtagagccagtagtcagtgctgatggcgatggtcatgaggccgaaggcggcgaaggcgcccaccgtcgtcagcagcacctgcacccccttctcgcaccagaggccccgctcttcgttccagcgcttcagcgactccagtttgaccacgggcagccggggggccgtgggccaccaccggggcagcgggggcggggccgtgccggcggctgggggggggttcacagcgcaggcagaagcggggggcccggggccggcggggctggggaggggggcggcgaggaggaggctgcggccggggagggggtcagagcgcggccatggtcggcggctggtggagggcaagg

SEQ ID NO: 14286 - RNA, 1809 nt, Homo sapiens
  source 1..1809: mol_type = other RNA
gctgggattacaggcatgagccaccgcgcccggccaggacaagttttacatcttgctctgttagggccctcagtgcttcatgtgaatcaagactgaaggcctctgaaagatatacttctccgaggagttagctgagataagcttattatccttttccttgtcttccatcttctttgcctctccaggctctgaagcaacctgagatgtcattaaggtgggggaagtacaaagttcttcagggttctgattgtggatgttttcattttctttggcctcaggagttcttactggcttctctggtggttctggattaggagagacctctagggaggtcctaggacttgcagtcccagtccccaaggaggccctagggctggtgggtgaaccccctccagaggctgtagggctggaaggtatgttccctgaggagggcctggggcttgcagtggctctgggtggaggaggcctactagggggtgctgaggtcctctggatagaggctctcttctttggttgttcagatccttcacttgcggtgcgggttcggaggactacttctgtggcagatgatgaaggctgccctgaagggctcagggctccgcctggtgatggagttgtggagctggggagaacttcctcctgggacttggccctttcagtggtaggagagggctgggcctgggcggggccattgcaggctggtagaggctcatcttcctcagaggagcttgcttcagatccttccttctctatttcctcctcttctaagagctccttgatctcagaattgtcttccccttgggctgcatcaggtgccagatcttcagttgctgagacagattcactctcactcttcaaggaaagtgtagagggactagtaggtgaggtaagaggactggagactgtagctgttcgaactgggggagaaatgactaaagagcgcctgctgctgcttgacagtcccttcaccacaaagactttattggaatgttgcttctccagtttgctcatcacctcgtagagattgtggttcagcttgctcatttccctgtagaagacatccctcaagttggaaatgttttggaagatggtcacatagcagccaatacgactattataaagaataggcagctcctctagtagttcttggttcagatcttcaaacacagtctgggctttgttgaactcttcctctgccttggcagtcttggcctcatctttcttcttggcattctgcactgcctccaggtggtgtcgggcactgtcatagtccacgagtttccgaccccgcttggcaattctctccttaatttcactgaactgggcaacatagatttccatggtccttacagcctggtcagccagtttctcctcgtagtcttcccaaaggagatcattattccatacgatggccttcagctcctcatgaccgtcccactcgctgctgtagatctcctgcagggtttctgacactctttttgaactttcatgcatcactttgactgcactaaggaagttcttcaggtccttgtacagcttgtggccttctgcctgttgttggtagaagttgctagcgctttgttcaaatcgttcatctttggtttctacagctttccccaatttctgcagcaccttctcctgggccctgctaaacttcttctgcacctgcttggcgaagaggccggccgcgccgcctgccttgccctctgccatcctgccaactccctgggggccgccgccctggccccgcgccctgtggttttctgaggcccccgaggaggaagtgcgggctcccggcatgcctcgcat

SEQ ID NO: 14287 - RNA, 878 nt, Homo sapiens
  source 1..878: mol_type = other RNA
gctgggattacaggcatgagccaccgcgcccggccatgagtgattttttgttgttgttgttctttttcatgatcttttttcctccttatctacagcgaccacacttgactcatagcagactcaaggttgtgggatgtgtcggatgctgcgtggcattcaagcacccacaggcaaggaggctgccaaggtcgagggctgcggagtcccagggcccatgagtccggccggagtctggtgtggacactctgaacacacgcagaggccttgtggcactcacctcagttacagccgaccacgcaggaatagattctgtacgtggtagagttgtctgttttcaccagcagtgtcttaaatactgtgcagttcccagtgggatcccatagtgtagaatcggtgggagccctgagctcattttcctgcaactggactgtcccatcttacagaagtgcctgtgagagattgtggtgaggtgcttggggcaggaaggtcctgggctgagcccagagcctgagcaagccctccgtgtgtggcgttcttcagcacatgatccagttaaaaagggacctgctgactgaaacttacattcatttttaacataaagttaccctggaaacgctggatccagaatggtggcagagggtgagccgtctcctctttaagtagctccctgtcctgctcccagcgcagggcgtgccacagtccttccaccttctcagcggggacaggaaccatctgggtcccctgggctcacagcatggaaagcaggctcagcccaagggtccgcattagtggctgcatcgtggctgtggccctgtgtcagctccgggcttgcactgccaggctggctgtagcgactctggctctctctggttgtccat

SEQ ID NO: 14288 - RNA, 737 nt, Homo sapiens
  source 1..737: mol_type = other RNA
gctgggattacaggcatgagccaccgcgcccggccatgagtgattttttgttgttgttgttctttttcatgatcttttttcctccttatctacagcgaccacacttgactcatagcagactcaaggttgtgggatgtgtcggatgctgcgtggcattcaagcacccacaggcaaggaggctgccaaggtcgagggctgcggagtcccagggcccatgagtccggccggagtctggtgtggacactctgaacacacgcagaggccttgtggcactcacctcagttacagccgaccacgcaggaatagattctgtacgtggtagagttgtctgttttcaccagcagtgtcttaaatactgtgcagttcccagtgggatcccatagtgtagaatcggtgggagccctgagctcattttcctgcaactggactgtcccatcttacattcatttttaacataaagttaccctggaaacgctggatccagaatggtggcagagggtgagccgtctcctctttaagtagctccctgtcctgctcccagcgcagggcgtgccacagtccttccaccttctcagcggggacaggaaccatctgggtcccctgggctcacagcatggaaagcaggctcagcccaagggtccgcattagtggctgcatcgtggctgtggccctgtgtcagctccgggcttgcactgccaggctggctgtagcgactctggctctctctggttgtccat

SEQ ID NO: 14289 - RNA, 679 nt, Homo sapiens
  source 1..679: mol_type = other RNA
gctgggattacaggcatgagccaccgcgcccggccatgagtgattttttgttgttgttgttctttttcatgatcttttttcctccttatctacagcgaccacacttgactcatagcagactcaaggttgtgggatgtgtcggatgctgcgtggcattcaagcacccacaggcaaggaggctgccaaggtcgagggctgcggagtcccagggcccatgagtccggccggagtctggtgtggacactctgaacacacgcagaggccttgtggcactcacctcagttacagccgaccacgcaggaatagattctgtacgtggtagagttgtctgttttcaccagcagtgtcttaaatactgtgcagttcccagtgggatcccttacattcatttttaacataaagttaccctggaaacgctggatccagaatggtggcagagggtgagccgtctcctctttaagtagctccctgtcctgctcccagcgcagggcgtgccacagtccttccaccttctcagcggggacaggaaccatctgggtcccctgggctcacagcatggaaagcaggctcagcccaagggtccgcattagtggctgcatcgtggctgtggccctgtgtcagctccgggcttgcactgccaggctggctgtagcgactctggctctctctggttgtccat

SEQ ID NO: 14290 - RNA, 1652 nt, Homo sapiens
  source 1..1652: mol_type = other RNA
gctgggattacaggcatgagccaccgcgcccggccatgagttgcttcttttaattaaaaattccttttccaggtgagtttgtgctactgtgtcagtctgtgtgtcagatcttgttgatctaggttatgctgttactttattacttctcgtgatggaaaaggcgtgttttgacaaggtcggtggaaagatgtaatacatcttggactctggaatatccatctagtaaaatggatgtgcagtatactgacaggggtggtgctgaggctctgaaggaaaggagtttgtaatttaagttgcttttaacaatttctcaagtaaatgtacacatcctgcctctgtcttggatttgtttttcatgcattggcttttatcacttatatttttcttttggatatgccaattaggtggcccagttcattgttttccgcccagagacgtgcacgatgcagtgctcaaatcagatatcccttctccttcggaaaaaatggttggatattacatacatggacacacctttctcagtcagaggacaaaagtaggaagtttttgattttgttcaagaagaaaatgtctggcaatttaggtcactcttcacaggaaaaattggctttaaaaacattaatcaaacgtgcactttgaaacactgctgctagtctgcccttcaaagaggagtgcatgttgagaaaaggcaatagtcgccccgttttctcacaaatctctaatctgagctggtccaggtgggagggctcaggtctgttctgcataccatcagctggggtgggtcgagtggaggctggggggtccaccttcaagacggctcactcacatgactggcagctgggagcttgggctgggggtgggtcatcagaagacccggggtgaggggagccctgtcttctgtccacgtgcacccctccatggcttgttggcttccacgcagcatggcggcggagttccaaaggtgaacatcaggggttgtaatatgctttatgtgagtaacttgggttgtgctttgaaaattttcaccctttgattaagggataagggtaggcccttaagctacatagttctttaaaatccatgtccctgactctggtgtcctctgtcacaggctacttaaagggctggtgtccatgggaggtattccagctcccaaagtgtgtggggtgcctaagttctcagcagagatgggaagttgagtcacagtgatgtgaactgaggtgatggtgggtaccccctgggtagagttgtcttggagaagcacagaatcaatcattaaataccattctctgtgacttaaaagtcaagtgctgggttttcaccactcccttgatcttgctcaaaaggaaacttaatcaagagaatgttgctgtactccgcttgcttcaaatgggttctgcgtggctaaggttacatttggtagctcttggcttgtcttcagtttcaaatgtagggtgagagaggatgttgtttggagagtcctctaagccctctctgctgatggaaagaacgtgtttcagtgcttattggcctcctaagtttctgagagttgtttttgagtcatttagaaataattaaactgggttaagcaaatgctttttgcttcagagcttcaacatttattagtcagttgtcctgtagagcaggttttt

SEQ ID NO: 14291 - RNA, 2063 nt, Homo sapiens
  source 1..2063: mol_type = other RNA
gctgggattacaggcatgagccaccgcgcccggccatgtttcttctttttcactgggtacttctgatattttccccaaattgattcaagtaatttgcagtcctaccatggatgtattggatttctacgtgagccctactacctctgacatttgatattgtcattttcatcatgtgaaatgaatacctcaacattgatccctctcttcaggaatgatcgacagatagtccagaaagcataggctgtagattttgttccagaacctcctgggatcatcagattgaacacatgagggtgggagactgccatacaagccatgagctcttttccgtgggtctcaactgggcattcacaacatagattggaagtaaggtggagacccaaaatttgtgatcagacatgattaccttccacagtgtgtggcctgaaatctcacccccctctggaggtcctagattgtcctccagagccttctgggatcatcagatctgtccctgaggctccaccacgctgaagggtgcattgtcctctccgctgttcacctcccggctgcatcttgggggtttctctggctgtgctgagcctcaaataacagaatcccgaggaacaccaggaccaagcctgccatgcccatgcggatgagattctccactgtgtaatccttggcgtgtgaggcaggtgtggagggcggccctgtgggtgggaggctggagcctccagagggtcctgagaccatgagctccaggggctcactggggtgagacagcaggtgggggttggagctgcgtgagccgtagcacctgtaggtccccgcgtgggctgaggtcacaggactcatggggaattcagcctggtacttatgagctccgtacattgatctcagacgcagtgggggatgggctgccccttctttggtcagaaggaaagtgtcaaaataaccccgtgactgacacagcagggtcacgttctctcctgaggccactgtggggcccggctgtgctgacagggagacggtgtcatagatctgtcctgccatcaggatgttcagggggtcgctgggggccgaccactcggaggagaggttgtgtgcaccatagcacctgtactggcccccgtgggaggggctcacagggcccagggtgaagttggcctgggagagcccagcctggggctgctggccagggcgctggaggaagtcacgttccccctccttatacagaacaaatctgtcgtagccgacatcagagccacactggagggtcaggctctgcccaggggccaggacagggccctgcagggtcaggagggagggcttcctagacacgcctgagggcagaatctccagggggtcactggggtgggaccacacccagggggtgtttgtataatagtaatagcatgtgaacctccacctgtggctgggggtcacggggcccacagggaacagggcctggaaccccccactgtggagctgctgtgagtccagggtccgggggagctggtgttctccttccttcatcagaacaaaatggtgatatcccttctgtgagccacatcggagggtcatattcccccctgaggccaccacagggctgggcagggctgagagggtgggtttgttgtagaatcctgtcatcaccagctccagggggtcgctgggctctgaccagcctgcagagctgtaatagtggcagcggtatctccctgcatggtgctgtgtcatggatgggatggagaatctggccttgttcttgggttccagtgggttatttctgtcccagggctctgggcttccctctttatccagttggtactcctgggcctccaggctcccctgacaccagatggtcacggggctcccccagctgatcacagagcctggctcagcccagagggtgggtttggggaagggccctgcctgcacgcgggtcctggggcccagactcagcccaaggcagagcagggctgtgagggcgggcgtcatggcgtctcctcccggtgacccggcgctctgcagagggatgagccctcagtgctggcaggacagagagacacacagggtgt

SEQ ID NO: 14292 - RNA, 2127 nt, Homo sapiens
  source 1..2127: mol_type = other RNA
gctgggattacaggcatgagccaccgcgcccggccatgtttcttctttttcactgggtacttctgatattttccccaaattgattcaagtaatttgcagtcctaccatggatgtattggatttctacgtgagccctactacctctgacatttgatattgtcattttcatcatgtgaaatgaatacctcaacattgatccctctcttcaggaatgatcgacagatagtccagaaagcataggctgtagattttgttccagaacctcctgggatcatcagattgaacacatgagggtgggagactgccatacaagctgggaaggaggaatcagatgatattgtcatgaattcctcaagagttagtgtttgctggcctccaagaggcaaggatctctgggaacttaagacagagaagcacttcacactcacccatgagctcttttccgtgggtctcaactgggcattcacaacatagattggaagtaaggtggagacccaaaatttgtgatcagacatgattaccttccacagtgtgtggcctgaaatctcacccccctctggaggtcctagattgtcctccagagccttctgggatcatcagatctgtccctgaggctccaccacgctgaagggtgcattgtcctctccgctgttcacctcccggctgcatcttgggggtttctctggctgtgctgagcctcaaataacagaatcccgaggaacaccaggaccaagcctgccatgcccatgcggatgagattctccactgtgtaatccttggcgtgtgaggctgagaccatgagctccaggggctcactggggtgagacagcaggtgggggttggagctgcgtgagccgtagcacctgtaggtccccgcgtgggctgaggtcacaggactcatggggaattcagcctggtacttatgagctccgtacattgatctcagacgcagtgggggatgggctgccccttctttggtcagaaggaaagtgtcaaaataaccccgtgactgacacagcagggtcacgttctctcctgaggccactgtggggcccggctgtgctgacagggagacggtgtcatagatctgtcctgccatcaggatgttcagggggtcgctgggggccgaccactcggaggagaggttgtgtgcaccatagcacctgtactggcccccgtgggaggggctcacagggcccagggtgaagttggcctgggagagcccagcctggggctgctggccagggcgctggaggaagtcacgttccccctccttatacagaacaaatctgtcgtagccgacatcagagccacactggagggtcaggctctgcccaggggccaggacagggccctgcagggtcaggagggagggcttcctagacacgcctgagggcagaatctccagggggtcactggggtgggaccacacccagggggtgtttgtataatagtaatagcatgtgaacctccacctgtggctgggggtcacggggcccacagggaacagggcctggaaccccccactgtggagctgctgtgagtccagggtccgggggagctggtgttctccttccttcatcagaacaaaatggtgatatcccttctgtgagccacatcggagggtcatattcccccctgaggccaccacagggctgggcagggctgagagggtgggtttgttgtagaatcctgtcatcaccagctccagggggtcgctgggctctgaccagcctgcagagctgtaatagtggcagcggtatctccctgcatggtgctgtgtcatggatgggatggagaatctggccttgttcttgggttccagtgggttatttctgtcccagggctctgggcttccctctttatccagttggtactcctgggcctccaggctcccctgacaccagatggtcacggggctcccccagctgatcacagagcctggctcagcccagagggtgggtttggggaagggccctgcctgcacgcgggtcctggggcccagactcagcccaaggcagagcagggctgtgagggcgggcgtcatggcgtctcctcccggtgacccggcgctctgcagagggatgagccctcagtgctggcaggacagagagacacacagggtgt

SEQ ID NO: 14293 - RNA, 3127 nt, Homo sapiens
  source 1..3127: mol_type = other RNA
gctgggattacaggcatgagccaccgcgcccggcccacaccagtttttaattagtgcttctcatctacaaatccagtcttcattacctgctcagtcaacgtggacatgagcctttttctccttcgccagtctgcacagtgctaattttgtcggtagagggtgctggagacattgcagaaggaaggggagaggcactctgctgcgggttctgagcgtccccgcccactactgattagctgggccatttctcagggttgtgtttgcagcgagaaatctccaggacaaagagcaggatagcctaccacttactataaaagcagtggatttcccaagctccgtggatttccacctgggatcctctgtcttgttccattttctttgctagtatttgctaccattttctttgtagttttttccctcattctcatcctctcggaggcctcatattctaggtgacggaagaatgatcccccatgcacaggttggaaatgttttattaaatacatttttggtaaagaagcctagtacaagatgccggctttagataatagggcagtctaatgacttctgaattcctcagataaggagttttgcctccagatggtctgcttgatggccaccaggtgatctttgctgtcctcaaaagtatgtgaaaatacctgggtccactcatttgtctggggatcataagcctccacagtattaaggtatgcctgtccatcataccccccaacagcatataacttatcaccaagtaaacagacccccactgcatctctgctgatgctcatggatgctactgcagtccacatgtctgttttgggatcatatctttccacacagtctgagagtctggaagtcaagttggatgcgggagcatcgtgcccccctatagcatacagcagtccattccaggtcgtcactcctacgccacctctcctttttgacatctgtgcacacagtgtccacttattagtatgaggatcaaaacattctactgatttgagacaagaacttccatcacgaccaccaactgcataaagttttccacttagtactgccacacctactgtactcctaggggtagacatagtggcaacaaaattccactggcgagcctgagggtcccatctttccactgtgttcagatagctccagccatcatgtcctcctacggcatacatgggaccttccagtacagccacaccaaggccatgtctatgtgtggacataggtggcatcacactccaagtttttgttttggggttgtagcactctacagtattcaaagtcttcagtccatctcttcctccaaccacatacagtttgtcatctagcactgcaacaccgaactgtagcctcctcccattcatatttgctactggagtccacatatttgtacggagatcatacttttcaatgcttgttgctccttttgttgaatccattcccccaactgcaaataatgtaccaacagttgacttcctaggttttgtccgaggactttgtaacatgggtcgtctctctggtaataaatggtacttcattgcttccataatgagtttctgacattctatatcatcccgaaaaagtacattattttccatgtctgccaggaactgtggtgcaagaagaggtagcctaatataagccaaaagtttacttagatctttccgtctctgttccaaatcatgacggacccaagtaagaagtgcattcaatattgtctcctcattaggaatgttcatgtcatcactagccaagagctttgcaatttcgctggctggtaataatacaaattcctggtttctgattacttccatgaaatgctccatagtataattgtgagccactttatgcaaatctgtacaaccttgggcatcagcaaaagaacgaattccaagacagttggatggatgaagctgtttcattaaaaacttacagcatgcttctacaacctgtgaaagctgaagaaggcaagctgtagataacaggcactcaatattatcttcttttaattcaaggcggcctgtataagcatactggatcaaggaccacaacgaatttggttctacaccttccatttttatttcttcttgtcttgcctctctgacatcattagtaaacatggcagcaaaatagtctgagacagaggagagcaccaatctgtgagctggaattctgcgatcaccagcgactaaaattacatcacacaactgtttatgtctcaaatagttttccatttttttaaatgtttgctcggcatgattaagggcttggaaaaattcatctgatgtacatggctccatagtatgacaggatgataatgtctgactactattggaagtcctgcatgaactggaatcagattcattttcttcttcactagtgccatcatccacttctggtctatccagccaatgtgcaccgccacaatcttctgctgtaaactcaaatgcagggacttcagaggtggatgccattggccaagaaggtgaattctgaaaatccagttggctggaccttcggtaaccaattgaagccaaaggcaattgtaggctacatggatctaaaaactttctcccaccgtttgctccagtctgtcctcggttccaaaattctccctgctggctgtcaactgtagaattaggagatgatgcttgatgaccaaaccacctccatctgattttcaaaatctgtttcacatcaaactctttacgagaaccagacatcctcagagaaaccaagtgatcgtctaggcaacgggcaaaaagcactgcacacagatttgtgcatccaaccaagacaagagaagtatatgccctgcgcgtcgggctccggaggcggccgtgggtcacggcgggccggggcggccaggcgggaggagcgggggaggcgggggccggggccggcgagctgagtgggatgctcggcccctcgcgcgcccctagaccctgtccgggcagcctcatccccggcgccggccggcccggagcgagccactcccgctccgtcaggcggcgccaggccggggggtcagagtccccgggtggccccggagggggcgggcgagtaggtgggggtaggggaccggttagcccgtcagtcccggcgcggcgcagtcggc

SEQ ID NO: 14294 - RNA, 2963 nt, Homo sapiens
  source 1..2963: mol_type = other RNA
gctgggattacaggcatgagccaccgcgcccggcccacaccagtttttaattagtgcttctcatctacaaatccagtcttcattacctgctcagtcaacgtggacatgagcctttttctccttcgccagtctgcacagtgctaattttgtcggtagagggtgctggagacattgcagaaggaaggggagaggcactctgctgcgggttctgagcgtccccgcccactactgattagctgggccatttctcagggttgtgtttgcagcgagaaatctccaggacaaagagcaggatagcctaccacttactataaaagcagtggatttcccaagctccgtggatttccacctgggatcctctgtcttgttccattttctttgctagtatttgctaccattttctttgtagttttttccctcattctcatcctctcggaggcctcatattctaggtgacggaagaatgatcccccatgcacaggttggaaatgttttctgggtccactcatttgtctggggatcataagcctccacagtattaaggtatgcctgtccatcataccccccaacagcatataacttatcaccaagtaaacagacccccactgcatctctgctgatgctcatggatgctactgcagtccacatgtctgttttgggatcatatctttccacacagtctgagagtctggaagtcaagttggatgcgggagcatcgtgcccccctatagcatacagcagtccattccaggtcgtcactcctacgccacctctcctttttgacatctgtgcacacagtgtccacttattagtatgaggatcaaaacattctactgatttgagacaagaacttccatcacgaccaccaactgcataaagttttccacttagtactgccacacctactgtactcctaggggtagacatagtggcaacaaaattccactggcgagcctgagggtcccatctttccactgtgttcagatagctccagccatcatgtcctcctacggcatacatgggaccttccagtacagccacaccaaggccatgtctatgtgtggacataggtggcatcacactccaagtttttgttttggggttgtagcactctacagtattcaaagtcttcagtccatctcttcctccaaccacatacagtttgtcatctagcactgcaacaccgaactgtagcctcctcccattcatatttgctactggagtccacatatttgtacggagatcatacttttcaatgcttgttgctccttttgttgaatccattcccccaactgcaaataatgtaccaacagttgacttcctaggttttgtccgaggactttgtaacatgggtcgtctctctggtaataaatggtacttcattgcttccataatgagtttctgacattctatatcatcccgaaaaagtacattattttccatgtctgccaggaactgtggtgcaagaagaggtagcctaatataagccaaaagtttacttagatctttccgtctctgttccaaatcatgacggacccaagtaagaagtgcattcaatattgtctcctcattaggaatgttcatgtcatcactagccaagagctttgcaatttcgctggctggtaataatacaaattcctggtttctgattacttccatgaaatgctccatagtataattgtgagccactttatgcaaatctgtacaaccttgggcatcagcaaaagaacgaattccaagacagttggatggatgaagctgtttcattaaaaacttacagcatgcttctacaacctgtgaaagctgaagaaggcaagctgtagataacaggcactcaatattatcttcttttaattcaaggcggcctgtataagcatactggatcaaggaccacaacgaatttggttctacaccttccatttttatttcttcttgtcttgcctctctgacatcattagtaaacatggcagcaaaatagtctgagacagaggagagcaccaatctgtgagctggaattctgcgatcaccagcgactaaaattacatcacacaactgtttatgtctcaaatagttttccatttttttaaatgtttgctcggcatgattaagggcttggaaaaattcatctgatgtacatggctccatagtatgacaggatgataatgtctgactactattggaagtcctgcatgaactggaatcagattcattttcttcttcactagtgccatcatccacttctggtctatccagccaatgtgcaccgccacaatcttctgctgtaaactcaaatgcagggacttcagaggtggatgccattggccaagaaggtgaattctgaaaatccagttggctggaccttcggtaaccaattgaagccaaaggcaattgtaggctacatggatctaaaaactttctcccaccgtttgctccagtctgtcctcggttccaaaattctccctgctggctgtcaactgtagaattaggagatgatgcttgatgaccaaaccacctccatctgattttcaaaatctgtttcacatcaaactctttacgagaaccagacatcctcagagaaaccaagtgatcgtctaggcaacgggcaaaaagcactgcacacagatttgtgcatccaaccaagacaagagaagtatatgccctgcgcgtcgggctccggaggcggccgtgggtcacggcgggccggggcggccaggcgggaggagcgggggaggcgggggccggggccggcgagctgagtgggatgctcggcccctcgcgcgcccctagaccctgtccgggcagcctcatccccggcgccggccggcccggagcgagccactcccgctccgtcaggcggcgccaggccggggggtcagagtccccgggtggccccggagggggcgggcgagtaggtgggggtaggggaccggttagcccgtcagtcccggcgcggcgcagtcggc

SEQ ID NO: 14295 - RNA, 4013 nt, Homo sapiens
  source 1..4013: mol_type = other RNA
gctgggattacaggcatgagccaccgcgcccggcccacaccagtttttaattagtgcttctcatctacaaatccagtcttcattacctgctcagtcaacgtggacatgagcctttttctccttcgccagtctgcacagtgctaattttgtcggtagagggtgctggagacattgcagaaggaaggggagaggcactctgctgcgggttctgagcgtccccgcccactactgattagctgggccatttctcagggttgtgtttgcagcgagaaatctccaggacaaagagcaggatagcctaccacttactataaaagcagtggatttcccaagctccgtggatttccacctgggatcctctgtcttgttcctgtgggaattgaagggcacagggaagtgaccccaacacgatattcctactgctttctgtgccttcagtaataaaatccttttccttcaacccatggatgtcttctgccagcatccatgaaaccataacaggtcagcttattagctccagtagggcaaaagcaaatctcagatcctgataaccagccaatcctttctgagtccaatcctctgttatgggacatgattatttatttaaaatcttccctgttcagattaccctgtgatttctgtctcccaactggactctgtctgatacatcacagcagcagacgcatcctccttaggtggctattcatagtccttagaattgtaaagcatttggctcccttcaatgacatgaaacttctaataatgggtttatgacttcctgctaatggctcatgctctcatttccattcatgactgctccactcagcatccctgctctctgctttattgacagcaacagccctctgcacccaagtcattaactatgccatcctttctaaaatgcccttcttttgtcctttcacagaacatatttaaaaagaaaatagaaaggcacttatgaaacctctctgtgtgtgtatccattcaggcacaccataggcagaattatatagcctgtttctactcactaaaagtaaaaacttaaaatgtagcacagatgtggtgaggatgtatcttggcatcaagtatgtatcatcctgtgtaatgtagacagcttaaactcacctccatgtagcaatcttgcaaagattttttaaaaggctctaaggtcatacagatctggttggttttgaaatttggctctgacatttactagctagtttgcgtatcattaactgggaatagtcatatctacttcatacagctgttgtaaaaattaaatgagttaacatacatatgaaatgcttacttagtacagtgtctgtcacatatcaagttgactcaacctccctatgttaaaataatcaaatgaacaagtctaaagcaatttaataaaatatgaatttttaactcaatttcacttaggtgcctccacagctaagatagtccctaattgttttcagacccagagaaaactttctcagaggctcttagagactttctcagggtggccctgacatgtggagctcaggccctcattcctcggtctttcaccccatgctctcttctttcaattactttcttatcattggaagctttaccttggcttaccattttctttgctagtatttgctaccattttctttgtagttttttccctcattctcatcctctcggaggcctcatattctaggtgacggaagaatgatcccccatgcacaggttggaaatgttttattaaatacatttttggtaaagaagcctagtacaagatgccggctttagataatagggcagtctaatgacttctgaattcctcagataaggagttttgcctccagatggtctgcttgatggccaccaggtgatctttgctgtcctcaaaagtatgtgaaaatacctgggtccactcatttgtctggggatcataagcctccacagtattaaggtatgcctgtccatcataccccccaacagcatataacttatcaccaagtaaacagacccccactgcatctctgctgatgctcatggatgctactgcagtccacatgtctgttttgggatcatatctttccacacagtctgagagtctggaagtcaagttggatgcgggagcatcgtgcccccctatagcatacagcagtccattccaggtcgtcactcctacgccacctctcctttttgacatctgtgcacacagtgtccacttattagtatgaggatcaaaacattctactgatttgagacaagaacttccatcacgaccaccaactgcataaagttttccacttagtactgccacacctactgtactcctaggggtagacatagtggcaacaaaattccactggcgagcctgagggtcccatctttccactgtgttcagatagctccagccatcatgtcctcctacggcatacatgggaccttccagtacagccacaccaaggccatgtctatgtgtggacataggtggcatcacactccaagtttttgttttggggttgtagcactctacagtattcaaagtcttcagtccatctcttcctccaaccacatacagtttgtcatctagcactgcaacaccgaactgtagcctcctcccattcatatttgctactggagtccacatatttgtacggagatcatacttttcaatgcttgttgctccttttgttgaatccattcccccaactgcaaataatgtaccaacagttgacttcctaggttttgtccgaggactttgtaacatgggtcgtctctctggtaataaatggtacttcattgcttccataatgagtttctgacattctatatcatcccgaaaaagtacattattttccatgtctgccaggaactgtggtgcaagaagaggtagcctaatataagccaaaagtttacttagatctttccgtctctgttccaaatcatgacggacccaagtaagaagtgcattcaatattgtctcctcattaggaatgttcatgtcatcactagccaagagctttgcaatttcgctggctggtaataatacaaattcctggtttctgattacttccatgaaatgctccatagtataattgtgagccactttatgcaaatctgtacaaccttgggcatcagcaaaagaacgaattccaagacagttggatggatgaagctgtttcattaaaaacttacagcatgcttctacaacctgtgaaagctgaagaaggcaagctgtagataacaggcactcaatattatcttcttttaattcaaggcggcctgtataagcatactggatcaaggaccacaacgaatttggttctacaccttccatttttatttcttcttgtcttgcctctctgacatcattagtaaacatggcagcaaaatagtctgagacagaggagagcaccaatctgtgagctggaattctgcgatcaccagcgactaaaattacatcacacaactgtttatgtctcaaatagttttccatttttttaaatgtttgctcggcatgattaagggcttggaaaaattcatctgatgtacatggctccatagtatgacaggatgataatgtctgactactattggaagtccgcgtcgggctccggaggcggccgtgggtcacggcgggccggggcggccaggcgggaggagcgggggaggcgggggccggggccggcgagctgagtgggatgctcggcccctcgcgcgcccctagaccctgtccgggcagcctcatccccggcgccggccggcccggagcgagccactcccgctccgtcaggcggcgccaggccggggggtcagagtccccgggtggccccggagggggcgggcgagtaggtgggggtaggggaccggttagcccgtcagtcccggcgcggcgcagtcggctgcccgccccgccccctcccgccaggccccgccccctcgccgggtcgcgcgcccggagaggccgcggccgccactgccccgccgggggtttctttgctctcctgcgcggcgtggggacggcc

SEQ ID NO: 14296 - RNA, 4368 nt, Homo sapiens
  source 1..4368: mol_type = other RNA
gctgggattacaggcatgagccaccgcgcccggcccacaccagtttttaattagtgcttctcatctacaaatccagtcttcattacctgctcagtcaacgtggacatgagcctttttctccttcgccagtctgcacagtgctaattttgtcggtagagggtgctggagacattgcagaaggaaggggagaggcactctgctgcgggttctgagcgtccccgcccactactgattagctgggccatttctcagggttgtgtttgcagcgagaaatctccaggacaaagagcaggatagcctaccacttactataaaagcagtggatttcccaagctccgtggatttccacctgggatcctctgtcttgttcctgtgggaattgaagggcacagggaagtgaccccaacacgatattcctactgctttctgtgccttcagtaataaaatccttttccttcaacccatggatgtcttctgccagcatccatgaaaccataacaggtcagcttattagctccagtagggcaaaagcaaatctcagatcctgataaccagccaatcctttctgagtccaatcctctgttatgggacatgattatttatttaaaatcttccctgttcagattaccctgtgatttctgtctcccaactggactctgtctgatacatcacagcagcagacgcatcctccttaggtggctattcatagtccttagaattgtaaagcatttggctcccttcaatgacatgaaacttctaataatgggtttatgacttcctgctaatggctcatgctctcatttccattcatgactgctccactcagcatccctgctctctgctttattgacagcaacagccctctgcacccaagtcattaactatgccatcctttctaaaatgcccttcttttgtcctttcacagaacatatttaaaaagaaaatagaaaggcacttatgaaacctctctgtgtgtgtatccattcaggcacaccataggcagaattatatagcctgtttctactcactaaaagtaaaaacttaaaatgtagcacagatgtggtgaggatgtatcttggcatcaagtatgtatcatcctgtgtaatgtagacagcttaaactcacctccatgtagcaatcttgcaaagattttttaaaaggctctaaggtcatacagatctggttggttttgaaatttggctctgacatttactagctagtttgcgtatcattaactgggaatagtcatatctacttcatacagctgttgtaaaaattaaatgagttaacatacatatgaaatgcttacttagtacagtgtctgtcacatatcaagttgactcaacctccctatgttaaaataatcaaatgaacaagtctaaagcaatttaataaaatatgaatttttaactcaatttcacttaggtgcctccacagctaagatagtccctaattgttttcagacccagagaaaactttctcagaggctcttagagactttctcagggtggccctgacatgtggagctcaggccctcattcctcggtctttcaccccatgctctcttctttcaattactttcttatcattggaagctttaccttggcttaccattttctttgctagtatttgctaccattttctttgtagttttttccctcattctcatcctctcggaggcctcatattctaggtgacggaagaatgatcccccatgcacaggttggaaatgttttattaaatacatttttggtaaagaagcctagtacaagatgccggctttagataatagggcagtctaatgacttctgaattcctcagataaggagttttgcctccagatggtctgcttgatggccaccaggtgatctttgctgtcctcaaaagtatgtgaaaatacctgggtccactcatttgtctggggatcataagcctccacagtattaaggtatgcctgtccatcataccccccaacagcatataacttatcaccaagtaaacagacccccactgcatctctgctgatgctcatggatgctactgcagtccacatgtctgttttgggatcatatctttccacacagtctgagagtctggaagtcaagttggatgcgggagcatcgtgcccccctatagcatacagcagtccattccaggtcgtcactcctacgccacctctcctttttgacatctgtgcacacagtgtccacttattagtatgaggatcaaaacattctactgatttgagacaagaacttccatcacgaccaccaactgcataaagttttccacttagtactgccacacctactgtactcctaggggtagacatagtggcaacaaaattccactggcgagcctgagggtcccatctttccactgtgttcagatagctccagccatcatgtcctcctacggcatacatgggaccttccagtacagccacaccaaggccatgtctatgtgtggacataggtggcatcacactccaagtttttgttttggggttgtagcactctacagtattcaaagtcttcagtccatctcttcctccaaccacatacagtttgtcatctagcactgcaacaccgaactgtagcctcctcccattcatatttgctactggagtccacatatttgtacggagatcatacttttcaatgcttgttgctccttttgttgaatccattcccccaactgcaaataatgtaccaacagttgacttcctaggttttgtccgaggactttgtaacatgggtcgtctctctggtaataaatggtacttcattgcttccataatgagtttctgacattctatatcatcccgaaaaagtacattattttccatgtctgccaggaactgtggtgcaagaagaggtagcctaatataagccaaaagtttacttagatctttccgtctctgttccaaatcatgacggacccaagtaagaagtgcattcaatattgtctcctcattaggaatgttcatgtcatcactagccaagagctttgcaatttcgctggctggtaataatacaaattcctggtttctgattacttccatgaaatgctccatagtataattgtgagccactttatgcaaatctgtacaaccttgggcatcagcaaaagaacgaattccaagacagttggatggatgaagctgtttcattaaaaacttacagcatgcttctacaacctgtgaaagctgaagaaggcaagctgtagataacaggcactcaatattatcttcttttaattcaaggcggcctgtataagcatactggatcaaggaccacaacgaatttggttctacaccttccatttttatttcttcttgtcttgcctctctgacatcattagtaaacatggcagcaaaatagtctgagacagaggagagcaccaatctgtgagctggaattctgcgatcaccagcgactaaaattacatcacacaactgtttatgtctcaaatagttttccatttttttaaatgtttgctcggcatgattaagggcttggaaaaattcatctgatgtacatggctccatagtatgacaggatgataatgtctgactactattggaagtcctgcatgaactggaatcagattcattttcttcttcactagtgccatcatccacttctggtctatccagccaatgtgcaccgccacaatcttctgctgtaaactcaaatgcagggacttcagaggtggatgccattggccaagaaggtgaattctgaaaatccagttggctggaccttcggtaaccaattgaagccaaaggcaattgtaggctacatggatctaaaaactttctcccaccgtttgctccagtctgtcctcggttccaaaattctccctgctggctgtcaactgtagaattaggagatgatgcttgatgaccaaaccacctccatctgattttcaaaatctgtttcacatcaaactctttacgagaaccagacatcctcagagaaaccaagtgatcgtctaggcaacgggcaaaaagcactgcacacagatttgtgcatccaaccaagacaagagaagtatatgccctgcgcgtcgggctccggaggcggccgtgggtcacggcgggccggggcggccaggcgggaggagcgggggaggcgggggccggggccggcgagctgagtgggatgctcggcccctcgcgcgcccctagaccctgtccgggcagcctcatccccggcgccggccggcccggagcgagccactcccgctccgtcaggcggcgccaggccggggggtcagagtccccgggtggccccggagggggcgggcgagtaggtgggggtaggggaccggttagcccgtcagtcccggcgcggcgcagtcggc

SEQ ID NO: 14297 - RNA, 4204 nt, Homo sapiens
  source 1..4204: mol_type = other RNA
gctgggattacaggcatgagccaccgcgcccggcccacaccagtttttaattagtgcttctcatctacaaatccagtcttcattacctgctcagtcaacgtggacatgagcctttttctccttcgccagtctgcacagtgctaattttgtcggtagagggtgctggagacattgcagaaggaaggggagaggcactctgctgcgggttctgagcgtccccgcccactactgattagctgggccatttctcagggttgtgtttgcagcgagaaatctccaggacaaagagcaggatagcctaccacttactataaaagcagtggatttcccaagctccgtggatttccacctgggatcctctgtcttgttcctgtgggaattgaagggcacagggaagtgaccccaacacgatattcctactgctttctgtgccttcagtaataaaatccttttccttcaacccatggatgtcttctgccagcatccatgaaaccataacaggtcagcttattagctccagtagggcaaaagcaaatctcagatcctgataaccagccaatcctttctgagtccaatcctctgttatgggacatgattatttatttaaaatcttccctgttcagattaccctgtgatttctgtctcccaactggactctgtctgatacatcacagcagcagacgcatcctccttaggtggctattcatagtccttagaattgtaaagcatttggctcccttcaatgacatgaaacttctaataatgggtttatgacttcctgctaatggctcatgctctcatttccattcatgactgctccactcagcatccctgctctctgctttattgacagcaacagccctctgcacccaagtcattaactatgccatcctttctaaaatgcccttcttttgtcctttcacagaacatatttaaaaagaaaatagaaaggcacttatgaaacctctctgtgtgtgtatccattcaggcacaccataggcagaattatatagcctgtttctactcactaaaagtaaaaacttaaaatgtagcacagatgtggtgaggatgtatcttggcatcaagtatgtatcatcctgtgtaatgtagacagcttaaactcacctccatgtagcaatcttgcaaagattttttaaaaggctctaaggtcatacagatctggttggttttgaaatttggctctgacatttactagctagtttgcgtatcattaactgggaatagtcatatctacttcatacagctgttgtaaaaattaaatgagttaacatacatatgaaatgcttacttagtacagtgtctgtcacatatcaagttgactcaacctccctatgttaaaataatcaaatgaacaagtctaaagcaatttaataaaatatgaatttttaactcaatttcacttaggtgcctccacagctaagatagtccctaattgttttcagacccagagaaaactttctcagaggctcttagagactttctcagggtggccctgacatgtggagctcaggccctcattcctcggtctttcaccccatgctctcttctttcaattactttcttatcattggaagctttaccttggcttaccattttctttgctagtatttgctaccattttctttgtagttttttccctcattctcatcctctcggaggcctcatattctaggtgacggaagaatgatcccccatgcacaggttggaaatgttttctgggtccactcatttgtctggggatcataagcctccacagtattaaggtatgcctgtccatcataccccccaacagcatataacttatcaccaagtaaacagacccccactgcatctctgctgatgctcatggatgctactgcagtccacatgtctgttttgggatcatatctttccacacagtctgagagtctggaagtcaagttggatgcgggagcatcgtgcccccctatagcatacagcagtccattccaggtcgtcactcctacgccacctctcctttttgacatctgtgcacacagtgtccacttattagtatgaggatcaaaacattctactgatttgagacaagaacttccatcacgaccaccaactgcataaagttttccacttagtactgccacacctactgtactcctaggggtagacatagtggcaacaaaattccactggcgagcctgagggtcccatctttccactgtgttcagatagctccagccatcatgtcctcctacggcatacatgggaccttccagtacagccacaccaaggccatgtctatgtgtggacataggtggcatcacactccaagtttttgttttggggttgtagcactctacagtattcaaagtcttcagtccatctcttcctccaaccacatacagtttgtcatctagcactgcaacaccgaactgtagcctcctcccattcatatttgctactggagtccacatatttgtacggagatcatacttttcaatgcttgttgctccttttgttgaatccattcccccaactgcaaataatgtaccaacagttgacttcctaggttttgtccgaggactttgtaacatgggtcgtctctctggtaataaatggtacttcattgcttccataatgagtttctgacattctatatcatcccgaaaaagtacattattttccatgtctgccaggaactgtggtgcaagaagaggtagcctaatataagccaaaagtttacttagatctttccgtctctgttccaaatcatgacggacccaagtaagaagtgcattcaatattgtctcctcattaggaatgttcatgtcatcactagccaagagctttgcaatttcgctggctggtaataatacaaattcctggtttctgattacttccatgaaatgctccatagtataattgtgagccactttatgcaaatctgtacaaccttgggcatcagcaaaagaacgaattccaagacagttggatggatgaagctgtttcattaaaaacttacagcatgcttctacaacctgtgaaagctgaagaaggcaagctgtagataacaggcactcaatattatcttcttttaattcaaggcggcctgtataagcatactggatcaaggaccacaacgaatttggttctacaccttccatttttatttcttcttgtcttgcctctctgacatcattagtaaacatggcagcaaaatagtctgagacagaggagagcaccaatctgtgagctggaattctgcgatcaccagcgactaaaattacatcacacaactgtttatgtctcaaatagttttccatttttttaaatgtttgctcggcatgattaagggcttggaaaaattcatctgatgtacatggctccatagtatgacaggatgataatgtctgactactattggaagtcctgcatgaactggaatcagattcattttcttcttcactagtgccatcatccacttctggtctatccagccaatgtgcaccgccacaatcttctgctgtaaactcaaatgcagggacttcagaggtggatgccattggccaagaaggtgaattctgaaaatccagttggctggaccttcggtaaccaattgaagccaaaggcaattgtaggctacatggatctaaaaactttctcccaccgtttgctccagtctgtcctcggttccaaaattctccctgctggctgtcaactgtagaattaggagatgatgcttgatgaccaaaccacctccatctgattttcaaaatctgtttcacatcaaactctttacgagaaccagacatcctcagagaaaccaagtgatcgtctaggcaacgggcaaaaagcactgcacacagatttgtgcatccaaccaagacaagagaagtatatgccctgcgcgtcgggctccggaggcggccgtgggtcacggcgggccggggcggccaggcgggaggagcgggggaggcgggggccggggccggcgagctgagtgggatgctcggcccctcgcgcgcccctagaccctgtccgggcagcctcatccccggcgccggccggcccggagcgagccactcccgctccgtcaggcggcgccaggccggggggtcagagtccccgggtggccccggagggggcgggcgagtaggtgggggtaggggaccggttagcccgtcagtcccggcgcggcgcagtcggc

SEQ ID NO: 14298 - RNA, 4271 nt, Homo sapiens
  source 1..4271: mol_type = other RNA
gctgggattacaggcatgagccaccgcgcccggcccattatttttaaatagttagaacatagtgaataagctataattgtagacactgaaaaacaagacaaagtgatcaaactaattatagcactgacaggatgcaaaatggaagacagaggtaggtctgcaaacagccacacaggtggaaattccaattgtaaatggttctctttgaaatactcagttttacataaatgcttatccagcagcacgtcataaaccacagggccaaaacaatttcttgtcacgtaaacatggcgttggtagctaaaactcaaatttagcaacaaataattgttttcataggactcataagataaccttaaattgttagatgcttttagggcattggctaattcagaattggctggtattataacagaacttaatttttgcaggcatttaaagattttcatgcattatgtacctgaaggttttgtctcttaattttctttgaaccacacctcttctccttattataagaaaaaccctcttagggtaagggaagtccaaattaactgtcctgaaattttgcattatatttaaaccataatatttgatttacttctgtcaaacaaaacactactatttgggttctcatttgtagattatttaaaaacatgtttttcctgttaattatcaatgcatttactatcacaaggattaaaaagatcacttcaggtggtggggatgtttcatgaaacaccatggtggggagtaggtagtgggcaggcagagtgacaatcagcttaacctcctttcacctagctgttctttagaaaaacaaaaataaaagtcaaattgctttcagttttcaagagtgaaaatggaggcacaagaaggatattcagatgtgcaagcaaattgcttcttttacatccttatattttcttttcttttcttttttttttttttttttttttttgagacggagtctcgctctgccaccatgcccggcctcacaaagtattttctaaaatataatttgctgtagagttcacagatgagcacttttcacattaggtgatatgcaaacaaatcactattggctcagcaggaaacagactttttgtacactctagttaacatgaagttttccaataaaacaaatgacagcgggagggggtagtgaggaattcaactctgtaatgtccacctagaatccaagtaggaaaaaaataaagctattgaaataatttagtaatatcctataggtcaccagtgatttccataaaatgctgcacagatacaaagtcttgagtatgttacttagtagctaaaaagagagccttgtgtgaggcacagctgacttggaacattaaagagcctggcttccctttctgctttccattctcccaacagaaaaaaaggtcttcaaagaattggccagtcttacagctcaccttggggtgtagatgactctccactgtggtgctaggcaattttattgaacaggtggccactggtggtgatggctgaaccactcattaaacaaattgctctaaatggcctcagtatcaaggtgtgctttctgtacccttaatctgactttaatcctgcagaacctcagtcttaccatgtttaacagcattgccatgtacgatatgcctttatcctacactgtatatatactctttatgcagaagtatatctaactgaaaagtataaaaatataatggtggaaaacaaatgaattaaaaaatgtatcacggccgatagcccaggtaactgcaggtgaaatgtagccagaagtcagaatcttggggcaaaatcaagtatagtcttatgggctgtgccttcaaatggtttagttttataccctcttaaggcagaatcaaagttctcttaatgttttggcaagtgtttttcttcctggaggttcataaaaataggtggaagaatcagtctaatggcttgttggcatgctaagggaaggatgtcaagttgacatccttggatacttggttaaaaactaaggctagtaggtgaagaaaaacaacagaatagtttttggttttaaatttgtacaaaggctacttattgaatactggaaaaaatgacaacagtgttttaccatctttgcataagaaaaaaatgattttccttttgaaactgtagctcaggatttaatcctgagtcacgtcatcatgtggtaaaaacaatctggattttacaataatttatataaagcaaaaaaagtcataaaaatgctaaatgatgcagagctacaaatatgatgaaacatgagcagaggggtcaaatcagatttttactccaggcaggtgttaagtttgtgaaaagtgatgcaatttgttatacattcaaatgcaaattagaactagctgccttacgatgagatttcactgtcatttttttagcaccctaatttttgtcggttctgtaggtttcaagtagcagaaacttacatctatttccttcagaaaattaaggagcagatattttaatatgctttatgtaaataggattctgataattttagctttagttaatgcaacacacttccctgggcacaaccatgacctctctgagaactggaaaatactgcataattttaaaaatcagagtgtaatgacattccctgacaacttcaaataagttatgtgaggaggatgaactatgggtagtctagaccaccagtcatatttgtctagccgtagaaacagtgacaacttaaagatctgcaaagatcagagcagagctggctgaaggtgcagcattctatacatgtcctcatggagcttcagaaaggttataagatgacccactcattctggttggctgtggccatagacagacaccataaatcctgggatgtggtcaagtactgaactgggggcaggtctgagcttgcttatgatcctccgactagccctggaacagatagtgaagaactacacagaatcccacagctagctctctctctttctctctctttttttacctttgagaaccatccatgagattaatacaatattaatcaaatctgacacagctgagtgctggctcacagctaactatctggatatggggttttgttggctcttagctgactgcattatttaatcaaatattaagaaaggtataattcacatgcaacccttggcaaaaagaaaagaaggttaatttcttataaccagcacaaactgttaacctgttaagaaaagcccaactgtttctgcatttgaggcatacacacacatcatctctgtttctttataaactggagcgtgaaaggaggagggggacaaataagataaagccatgagctaaacacccagcaggccctactccttattctctgtgtgggtggcagcattagtcagaaagtcactcctctgctgtgatggtcatgacatatttgaacttgtagatctttaaggatttccttatttattctgccaggtctatggtaggtgcttgtttgttttcttggtggaatgattcatcaatgcttcctgagaggctcaaacaggatcactggccagattccaaagagaaacttcacttttggcctatatctcaggtaaagtgttcttgtatacaaactgaaaaggatgtgaagataggaaccaaggccagttaaaatatgccaccatgcatgaaattgtgtggtaatacctatgataggtggtaccttctttcgaaagttccatgtaacaatataaatagatcgaagtactaatgtaaagaccaacattccatacatgacctgatggaatatcggctcttttaccttaaggtaaactgtggttactattaaactgaatagaactaaggtaaaaagcagatggtagtttactgagttcttgatcttgaaacattcaaacatgcagtacacaaatatgcaacagctgtatatcattgggagttcatccaatagctgcatttcatatttcagagtcatgtggaagcaccaggatcccattcctaccactgtgagtgctaaataagaagcaatgtaccgcttttccagaccgtctctaacactctgaactgcaccgaacattggaggtataatcatgatcaggttactcactgtattccagaactcggcgatgtaccaggtcacggagtagttctcctcgcaccagtccagcgtggaggtcgtggggccccagtagccctctcggtccgcggccggagccatcacgccgccgccgccgccgcccaggcgctccgctcactgtgccgggttaggctggcgaccaggccggctc

SEQ ID NO: 14299 - RNA, 4419 nt, Homo sapiens
  source 1..4419: mol_type = other RNA
gctgggattacaggcatgagccaccgcgcccggcccattatttttaaatagttagaacatagtgaataagctataattgtagacactgaaaaacaagacaaagtgatcaaactaattatagcactgacaggatgcaaaatggaagacagaggtaggtctgcaaacagccacacaggtggaaattccaattgtaaatggttctctttgaaatactcagttttacataaatgcttatccagcagcacgtcataaaccacagggccaaaacaatttcttgtcacgtaaacatggcgttggtagctaaaactcaaatttagcaacaaataattgttttcataggactcataagataaccttaaattgttagatgcttttagggcattggctaattcagaattggctggtattataacagaacttaatttttgcaggcatttaaagattttcatgcattatgtacctgaaggttttgtctcttaattttctttgaaccacacctcttctccttattataagaaaaaccctcttagggtaagggaagtccaaattaactgtcctgaaattttgcattatatttaaaccataatatttgatttacttctgtcaaacaaaacactactatttgggttctcatttgtagattatttaaaaacatgtttttcctgttaattatcaatgcatttactatcacaaggattaaaaagatcacttcaggtggtggggatgtttcatgaaacaccatggtggggagtaggtagtgggcaggcagagtgacaatcagcttaacctcctttcacctagctgttctttagaaaaacaaaaataaaagtcaaattgctttcagttttcaagagtgaaaatggaggcacaagaaggatattcagatgtgcaagcaaattgcttcttttacatccttatattttcttttcttttcttttttttttttttttttttttttgagacggagtctcgctctgccaccatgcccggcctcacaaagtattttctaaaatataatttgctgtagagttcacagatgagcacttttcacattaggtgatatgcaaacaaatcactattggctcagcaggaaacagactttttgtacactctagttaacatgaagttttccaataaaacaaatgacagcgggagggggtagtgaggaattcaactctgtaatgtccacctagaatccaagtaggaaaaaaataaagctattgaaataatttagtaatatcctataggtcaccagtgatttccataaaatgctgcacagatacaaagtcttgagtatgttacttagtagctaaaaagagagccttgtgtgaggcacagctgacttggaacattaaagagcctggcttccctttctgctttccattctcccaacagaaaaaaaggtcttcaaagaattggccagtcttacagctcaccttggggtgtagatgactctccactgtggtgctaggcaattttattgaacaggtggccactggtggtgatggctgaaccactcattaaacaaattgctctaaatggcctcagtatcaaggtgtgctttctgtacccttaatctgactttaatcctgcagaacctcagtcttaccatgtttaacagcattgccatgtacgatatgcctttatcctacactgtatatatactctttatgcagaagtatatctaactgaaaagtataaaaatataatggtggaaaacaaatgaattaaaaaatgtatcacggccgatagcccaggtaactgcaggtgaaatgtagccagaagtcagaatcttggggcaaaatcaagtatagtcttatgggctgtgccttcaaatggtttagttttataccctcttaaggcagaatcaaagttctcttaatgttttggcaagtgtttttcttcctggaggttcataaaaataggtggaagaatcagtctaatggcttgttggcatgctaagggaaggatgtcaagttgacatccttggatacttggttaaaaactaaggctagtaggtgaagaaaaacaacagaatagtttttggttttaaatttgtacaaaggctacttattgaatactggaaaaaatgacaacagtgttttaccatctttgcataagaaaaaaatgattttccttttgaaactgtagctcaggatttaatcctgagtcacgtcatcatgtggtaaaaacaatctggattttacaataatttatataaagcaaaaaaagtcataaaaatgctaaatgatgcagagctacaaatatgatgaaacatgagcagaggggtcaaatcagatttttactccaggcaggtgttaagtttgtgaaaagtgatgcaatttgttatacattcaaatgcaaattagaactagctgccttacgatgagatttcactgtcatttttttagcaccctaatttttgtcggttctgtaggtttcaagtagcagaaacttacatctatttccttcagaaaattaaggagcagatattttaatatgctttatgtaaataggattctgataattttagctttagttaatgcaacacacttccctgggcacaaccatgacctctctgagaactggaaaatactgcataattttaaaaatcagagtgtaatgacattccctgacaacttcaaataagttatgtgaggaggatgaactatgggtagtctagaccaccagtcatatttgtctagccgtagaaacagtgacaacttaaagatctgcaaagatcagagcagagctggctgaaggtgcagcattctatacatgtcctcatggagcttcagaaaggttataagatgacccactcattctggttggctgtggccatagacagacaccataaatcctgggatgtggtcaagtactgaactgggggcaggtctgagcttgcttatgatcctccgactagccctggaacagatagtgaagaactacacagaatcccacagctagctctctctctttctctctctttttttacctttgagaaccatccatgagattaatacaatattaatcaaatctgacacagctgagtgctggctcacagctaactatctggatatggggttttgttggctcttagctgactgcattatttaatcaaatattaagaaaggtataattcacatgcaacccttggcaaaaagaaaagaaggttaatttcttataaccagcacaaactgttaacctgttaagaaaagcccaactgtttctgcatttgaggcatacacacacatcatctctgtttctttataaactggagcgtgaaaggaggagggggacaaataagataaagccatgagctaaacacccagcaggccctactccttattctctgtgtgggtggcagcattagtcagaaagtcactcctctgctgtgatggtcatgacatatttgaacttgtagatctttaaggatttccttatttattctgccaggtctatggtaggtgcttgtttgttttcttggtggaatgattcatcaatgcttcctgagaggctcaaacaggatcactggccagattccaaagagaaacttcacttttggcctatatctcaggtaaagtgttcttgtatacaaactgaaaaggatgtgaagataggaaccaaggccagttaaaatatgccaccatgcatgaaattgtgtggtaatacctatgataggtggtaccttctttcgaaagttcctcagtgactcacaaaatatgttatctatattccaaaataaaaatcccaataaaaatatacccaatgatgtataacccagtcctctaagccatggataaacccatggccaatcttcagctctcaggggcagttcaaagcaatactcttcatgtaacaatataaatagatcgaagtactaatgtaaagaccaacattccatacatgacctgatggaatatcggctcttttaccttaaggtaaactgtggttactattaaactgaatagaactaaggtaaaaagcagatggtagtttactgagttcttgatcttgaaacattcaaacatgcagtacacaaatatgcaacagctgtatatcattgggagttcatccaatagctgcatttcatatttcagagtcatgtggaagcaccaggatcccattcctaccactgtgagtgctaaataagaagcaatgtaccgcttttccagaccgtctctaacactctgaactgcaccgaacattggaggtataatcatgatcaggttactcactgtattccagaactcggcgatgtaccaggtcacggagtagttctcctcgcaccagtccagcgtggaggtcgtggggccccagtagccctctcggtccgcggccggagccatcacgccgccgccgccgccgcccaggcgctccgctcactgtgccgggttaggctggcgaccaggccggctc

SEQ ID NO: 14300 - RNA, 4251 nt, Homo sapiens
  source 1..4251: mol_type = other RNA
gctgggattacaggcatgagccaccgcgcccggcccattatttttaaatagttagaacatagtgaataagctataattgtagacactgaaaaacaagacaaagtgatcaaactaattatagcactgacaggatgcaaaatggaagacagaggtaggtctgcaaacagccacacaggtggaaattccaattgtaaatggttctctttgaaatactcagttttacataaatgcttatccagcagcacgtcataaaccacagggccaaaacaatttcttgtcacgtaaacatggcgttggtagctaaaactcaaatttagcaacaaataattgttttcataggactcataagataaccttaaattgttagatgcttttagggcattggctaattcagaattggctggtattataacagaacttaatttttgcaggcatttaaagattttcatgcattatgtacctgaaggttttgtctcttaattttctttgaaccacacctcttctccttattataagaaaaaccctcttagggtaagggaagtccaaattaactgtcctgaaattttgcattatatttaaaccataatatttgatttacttctgtcaaacaaaacactactatttgggttctcatttgtagattatttaaaaacatgtttttcctgttaattatcaatgcatttactatcacaaggattaaaaagatcacttcaggtggtggggatgtttcatgaaacaccatggtggggagtaggtagtgggcaggcagagtgacaatcagcttaacctcctttcacctagctgttctttagaaaaacaaaaataaaagtcaaattgctttcagttttcaagagtgaaaatggaggcacaagaaggatattcagatgtgcaagcaaattgcttcttttacatccttatattttcttttcttttcttttttttttttttttttttttttgagacggagtctcgctctgccaccatgcccggcctcacaaagtattttctaaaatataatttgctgtagagttcacagatgagcacttttcacattaggtgatatgcaaacaaatcactattggctcagcaggaaacagactttttgtacactctagttaacatgaagttttccaataaaacaaatgacagcgggagggggtagtgaggaattcaactctgtaatgtccacctagaatccaagtaggaaaaaaataaagctattgaaataatttagtaatatcctataggtcaccagtgatttccataaaatgctgcacagatacaaagtcttgagtatgttacttagtagctaaaaagagagccttgtgtgaggcacagctgacttggaacattaaagagcctggcttccctttctgctttccattctcccaacagaaaaaaaggtcttcaaagaattggccagtcttacagctcaccttggggtgtagatgactctccactgtggtgctaggcaattttattgaacaggtggccactggtggtgatggctgaaccactcattaaacaaattgctctaaatggcctcagtatcaaggtgtgctttctgtacccttaatctgactttaatcctgcagaacctcagtcttaccatgtttaacagcattgccatgtacgatatgcctttatcctacactgtatatatactctttatgcagaagtatatctaactgaaaagtataaaaatataatggtggaaaacaaatgaattaaaaaatgtatcacggccgatagcccaggtaactgcaggtgaaatgtagccagaagtcagaatcttggggcaaaatcaagtatagtcttatgggctgtgccttcaaatggtttagttttataccctcttaaggcagaatcaaagttctcttaatgttttggcaagtgtttttcttcctggaggttcataaaaataggtggaagaatcagtctaatggcttgttggcatgctaagggaaggatgtcaagttgacatccttggatacttggttaaaaactaaggctagtaggtgaagaaaaacaacagaatagtttttggttttaaatttgtacaaaggctacttattgaatactggaaaaaatgacaacagtgttttaccatctttgcataagaaaaaaatgattttccttttgaaactgtagctcaggatttaatcctgagtcacgtcatcatgtggtaaaaacaatctggattttacaataatttatataaagcaaaaaaagtcataaaaatgctaaatgatgcagagctacaaatatgatgaaacatgagcagaggggtcaaatcagatttttactccaggcaggtgttaagtttgtgaaaagtgatgcaatttgttatacattcaaatgcaaattagaactagctgccttacgatgagatttcactgtcatttttttagcaccctaatttttgtcggttctgtaggtttcaagtagcagaaacttacatctatttccttcagaaaattaaggagcagatattttaatatgctttatgtaaataggattctgataattttagctttagttaatgcaacacacttccctgggcacaaccatgacctctctgagaactggaaaatactgcataattttaaaaatcagagtgtaatgacattccctgacaacttcaaataagttatgtgaggaggatgaactatgggtagtctagaccaccagtcatatttgtctagccgtagaaacagtgacaacttaaagatctgcaaagatcagagcagagctggctgaaggtgcagcattctatacatgtcctcatggagcttcagaaaggttataagatgacccactcattctggttggctgtggccatagacagacaccataaatcctgggatgtggtcaagtactgaactgggggcaggtctgagcttgcttatgatcctccgactagccctggaacagatagtgaagaactacacagaatcccacagctagctctctctctttctctctctttttttacctttgagaaccatccatgagattaatacaatattaatcaaatctgacacagctgagtgctggctcacagctaactatctggatatggggttttgttggctcttagctgactgcattatttaatcaaatattaagaaaggtataattcacatgcaacccttggcaaaaagaaaagaaggttaatttcttataaccagcacaaactgttaacctgttaagaaaagcccaactgtttctgcatttgaggcatacacacacatcatctctgtttctttataaactggagcgtgaaaggaggagggggacaaataagataaagccatgagctaaacacccagcaggccctactccttattctctgtgtgggtggcagcattagtcagaaagtcactcctctgctgtgatggtcatgacatatttgaacttgtagatctttaaggatttccttatttattctgccaggtctatggtaggtgcttgtttgttttcttggtggaatgattcatcaatgcttcctgagaggctcaaacaggatcactggccagattccaaagagaaacttcacttttggcctatatctcaggtaaagtgttcttgtatacaaactgaaaaggatgtgaagataggaaccaaggccagttaaaatatgccaccatgcatgaaattgtgtggtaatacctatgataggtggtaccttctttcgaaagttcctcagtgactcacaaaatatgttatctatattccaaaataaaaatcccaataaaaatatacccaatgatgtataacccagtcctctaagccatggataaacccatgtaacaatataaatagatcgaagtactaatgtaaagaccaacattccatacatgacctgatggaatatcggctcttttaccttaaggtaaactgtggttactattaaactgaatagaactaaggtaaaaagcagatggtagtttactgagttcttgatcttgaaacattcaaacatgcagtacacaaatatgcaacagctgtatatcattgggagttcatccaatagctgcatttcatatttcagagtcatgtggaagcaccaggatcccattcctaccaagaactcggcgatgtaccaggtcacggagtagttctcctcgcaccagtccagcgtggaggtcgtggggccccagtagccctctcggtccgcggccggagccatcacgccgccgccgccgccgcccaggcgctccgctcactgtgccgggttaggctggcgac

SEQ ID NO: 14301 - RNA, 4362 nt, Homo sapiens
  source 1..4362: mol_type = other RNA
gctgggattacaggcatgagccaccgcgcccggcccattatttttaaatagttagaacatagtgaataagctataattgtagacactgaaaaacaagacaaagtgatcaaactaattatagcactgacaggatgcaaaatggaagacagaggtaggtctgcaaacagccacacaggtggaaattccaattgtaaatggttctctttgaaatactcagttttacataaatgcttatccagcagcacgtcataaaccacagggccaaaacaatttcttgtcacgtaaacatggcgttggtagctaaaactcaaatttagcaacaaataattgttttcataggactcataagataaccttaaattgttagatgcttttagggcattggctaattcagaattggctggtattataacagaacttaatttttgcaggcatttaaagattttcatgcattatgtacctgaaggttttgtctcttaattttctttgaaccacacctcttctccttattataagaaaaaccctcttagggtaagggaagtccaaattaactgtcctgaaattttgcattatatttaaaccataatatttgatttacttctgtcaaacaaaacactactatttgggttctcatttgtagattatttaaaaacatgtttttcctgttaattatcaatgcatttactatcacaaggattaaaaagatcacttcaggtggtggggatgtttcatgaaacaccatggtggggagtaggtagtgggcaggcagagtgacaatcagcttaacctcctttcacctagctgttctttagaaaaacaaaaataaaagtcaaattgctttcagttttcaagagtgaaaatggaggcacaagaaggatattcagatgtgcaagcaaattgcttcttttacatccttatattttcttttcttttcttttttttttttttttttttttttgagacggagtctcgctctgccaccatgcccggcctcacaaagtattttctaaaatataatttgctgtagagttcacagatgagcacttttcacattaggtgatatgcaaacaaatcactattggctcagcaggaaacagactttttgtacactctagttaacatgaagttttccaataaaacaaatgacagcgggagggggtagtgaggaattcaactctgtaatgtccacctagaatccaagtaggaaaaaaataaagctattgaaataatttagtaatatcctataggtcaccagtgatttccataaaatgctgcacagatacaaagtcttgagtatgttacttagtagctaaaaagagagccttgtgtgaggcacagctgacttggaacattaaagagcctggcttccctttctgctttccattctcccaacagaaaaaaaggtcttcaaagaattggccagtcttacagctcaccttggggtgtagatgactctccactgtggtgctaggcaattttattgaacaggtggccactggtggtgatggctgaaccactcattaaacaaattgctctaaatggcctcagtatcaaggtgtgctttctgtacccttaatctgactttaatcctgcagaacctcagtcttaccatgtttaacagcattgccatgtacgatatgcctttatcctacactgtatatatactctttatgcagaagtatatctaactgaaaagtataaaaatataatggtggaaaacaaatgaattaaaaaatgtatcacggccgatagcccaggtaactgcaggtgaaatgtagccagaagtcagaatcttggggcaaaatcaagtatagtcttatgggctgtgccttcaaatggtttagttttataccctcttaaggcagaatcaaagttctcttaatgttttggcaagtgtttttcttcctggaggttcataaaaataggtggaagaatcagtctaatggcttgttggcatgctaagggaaggatgtcaagttgacatccttggatacttggttaaaaactaaggctagtaggtgaagaaaaacaacagaatagtttttggttttaaatttgtacaaaggctacttattgaatactggaaaaaatgacaacagtgttttaccatctttgcataagaaaaaaatgattttccttttgaaactgtagctcaggatttaatcctgagtcacgtcatcatgtggtaaaaacaatctggattttacaataatttatataaagcaaaaaaagtcataaaaatgctaaatgatgcagagctacaaatatgatgaaacatgagcagaggggtcaaatcagatttttactccaggcaggtgttaagtttgtgaaaagtgatgcaatttgttatacattcaaatgcaaattagaactagctgccttacgatgagatttcactgtcatttttttagcaccctaatttttgtcggttctgtaggtttcaagtagcagaaacttacatctatttccttcagaaaattaaggagcagatattttaatatgctttatgtaaataggattctgataattttagctttagttaatgcaacacacttccctgggcacaaccatgacctctctgagaactggaaaatactgcataattttaaaaatcagagtgtaatgacattccctgacaacttcaaataagttatgtgaggaggatgaactatgggtagtctagaccaccagtcatatttgtctagccgtagaaacagtgacaacttaaagatctgcaaagatcagagcagagctggctgaaggtgcagcattctatacatgtcctcatggagcttcagaaaggttataagatgacccactcattctggttggctgtggccatagacagacaccataaatcctgggatgtggtcaagtactgaactgggggcaggtctgagcttgcttatgatcctccgactagccctggaacagatagtgaagaactacacagaatcccacagctagctctctctctttctctctctttttttacctttgagaaccatccatgagattaatacaatattaatcaaatctgacacagctgagtgctggctcacagctaactatctggatatggggttttgttggctcttagctgactgcattatttaatcaaatattaagaaaggtataattcacatgcaacccttggcaaaaagaaaagaaggttaatttcttataaccagcacaaactgttaacctgttaagaaaagcccaactgtttctgcatttgaggcatacacacacatcatctctgtttctttataaactggagcgtgaaaggaggagggggacaaataagataaagccatgagctaaacacccagcaggccctactccttattctctgtgtgggtggcagcattagtcagaaagtcactcctctgctgtgatggtcatgacatatttgaacttgtagatctttaaggatttccttatttattctgccaggtctatggtaggtgcttgtttgttttcttggtggaatgattcatcaatgcttcctgagaggctcaaacaggatcactggccagattccaaagagaaacttcacttttggcctatatctcaggtaaagtgttcttgtatacaaactgaaaaggatgtgaagataggaaccaaggccagttaaaatatgccaccatgcatgaaattgtgtggtaatacctatgataggtggtaccttctttcgaaagttcctcagtgactcacaaaatatgttatctatattccaaaataaaaatcccaataaaaatatacccaatgatgtataacccagtcctctaagccatggataaacccatgtaacaatataaatagatcgaagtactaatgtaaagaccaacattccatacatgacctgatggaatatcggctcttttaccttaaggtaaactgtggttactattaaactgaatagaactaaggtaaaaagcagatggtagtttactgagttcttgatcttgaaacattcaaacatgcagtacacaaatatgcaacagctgtatatcattgggagttcatccaatagctgcatttcatatttcagagtcatgtggaagcaccaggatcccattcctaccactgtgagtgctaaataagaagcaatgtaccgcttttccagaccgtctctaacactctgaactgcaccgaacattggaggtataatcatgatcaggttactcactgtattccagaactcggcgatgtaccaggtcacggagtagttctcctcgcaccagtccagcgtggaggtcgtggggccccagtagccctctcggtccgcggccggagccatcacgccgccgccgccgccgcccaggcgctccgctcactgtgccgggttaggctggcgac

SEQ ID NO: 14302 - RNA, 4343 nt, Homo sapiens
  source 1..4343: mol_type = other RNA
gctgggattacaggcatgagccaccgcgcccggcccattatttttaaatagttagaacatagtgaataagctataattgtagacactgaaaaacaagacaaagtgatcaaactaattatagcactgacaggatgcaaaatggaagacagaggtaggtctgcaaacagccacacaggtggaaattccaattgtaaatggttctctttgaaatactcagttttacataaatgcttatccagcagcacgtcataaaccacagggccaaaacaatttcttgtcacgtaaacatggcgttggtagctaaaactcaaatttagcaacaaataattgttttcataggactcataagataaccttaaattgttagatgcttttagggcattggctaattcagaattggctggtattataacagaacttaatttttgcaggcatttaaagattttcatgcattatgtacctgaaggttttgtctcttaattttctttgaaccacacctcttctccttattataagaaaaaccctcttagggtaagggaagtccaaattaactgtcctgaaattttgcattatatttaaaccataatatttgatttacttctgtcaaacaaaacactactatttgggttctcatttgtagattatttaaaaacatgtttttcctgttaattatcaatgcatttactatcacaaggattaaaaagatcacttcaggtggtggggatgtttcatgaaacaccatggtggggagtaggtagtgggcaggcagagtgacaatcagcttaacctcctttcacctagctgttctttagaaaaacaaaaataaaagtcaaattgctttcagttttcaagagtgaaaatggaggcacaagaaggatattcagatgtgcaagcaaattgcttcttttacatccttatattttcttttcttttcttttttttttttttttttttttttgagacggagtctcgctctgccaccatgcccggcctcacaaagtattttctaaaatataatttgctgtagagttcacagatgagcacttttcacattaggtgatatgcaaacaaatcactattggctcagcaggaaacagactttttgtacactctagttaacatgaagttttccaataaaacaaatgacagcgggagggggtagtgaggaattcaactctgtaatgtccacctagaatccaagtaggaaaaaaataaagctattgaaataatttagtaatatcctataggtcaccagtgatttccataaaatgctgcacagatacaaagtcttgagtatgttacttagtagctaaaaagagagccttgtgtgaggcacagctgacttggaacattaaagagcctggcttccctttctgctttccattctcccaacagaaaaaaaggtcttcaaagaattggccagtcttacagctcaccttggggtgtagatgactctccactgtggtgctaggcaattttattgaacaggtggccactggtggtgatggctgaaccactcattaaacaaattgctctaaatggcctcagtatcaaggtgtgctttctgtacccttaatctgactttaatcctgcagaacctcagtcttaccatgtttaacagcattgccatgtacgatatgcctttatcctacactgtatatatactctttatgcagaagtatatctaactgaaaagtataaaaatataatggtggaaaacaaatgaattaaaaaatgtatcacggccgatagcccaggtaactgcaggtgaaatgtagccagaagtcagaatcttggggcaaaatcaagtatagtcttatgggctgtgccttcaaatggtttagttttataccctcttaaggcagaatcaaagttctcttaatgttttggcaagtgtttttcttcctggaggttcataaaaataggtggaagaatcagtctaatggcttgttggcatgctaagggaaggatgtcaagttgacatccttggatacttggttaaaaactaaggctagtaggtgaagaaaaacaacagaatagtttttggttttaaatttgtacaaaggctacttattgaatactggaaaaaatgacaacagtgttttaccatctttgcataagaaaaaaatgattttccttttgaaactgtagctcaggatttaatcctgagtcacgtcatcatgtggtaaaaacaatctggattttacaataatttatataaagcaaaaaaagtcataaaaatgctaaatgatgcagagctacaaatatgatgaaacatgagcagaggggtcaaatcagatttttactccaggcaggtgttaagtttgtgaaaagtgatgcaatttgttatacattcaaatgcaaattagaactagctgccttacgatgagatttcactgtcatttttttagcaccctaatttttgtcggttctgtaggtttcaagtagcagaaacttacatctatttccttcagaaaattaaggagcagatattttaatatgctttatgtaaataggattctgataattttagctttagttaatgcaacacacttccctgggcacaaccatgacctctctgagaactggaaaatactgcataattttaaaaatcagagtgtaatgacattccctgacaacttcaaataagttatgtgaggaggatgaactatgggtagtctagaccaccagtcatatttgtctagccgtagaaacagtgacaacttaaagatctgcaaagatcagagcagagctggctgaaggtgcagcattctatacatgtcctcatggagcttcagaaaggttataagatgacccactcattctggttggctgtggccatagacagacaccataaatcctgggatgtggtcaagtactgaactgggggcaggtctgagcttgcttatgatcctccgactagccctggaacagatagtgaagaactacacagaatcccacagctagctctctctctttctctctctttttttacctttgagaaccatccatgagattaatacaatattaatcaaatctgacacagctgagtgctggctcacagctaactatctggatatggggttttgttggctcttagctgactgcattatttaatcaaatattaagaaaggtataattcacatgcaacccttggcaaaaagaaaagaaggttaatttcttataaccagcacaaactgttaacctgttaagaaaagcccaactgtttctgcatttgaggcatacacacacatcatctctgtttctttataaactggagcgtgaaaggaggagggggacaaataagataaagccatgagctaaacacccagcaggccctactccttattctctgtgtgggtggcagcattagtcagaaagtcactcctctgctgtgatggtcatgacatatttgaacttgtagatctttaaggatttccttatttattctgccaggtctatggtaggtgcttgtttgttttcttggtggaatgattcatcaatgcttcctgagaggctcaaacaggatcactggccagattccaaagagaaacttcacttttggcctatatctcaggtaaagtgttcttgtatacaaactgaaaaggatgtgaagataggaaccaaggccagttaaaatatgccaccatgcatgaaattgtgtggtaatacctatgataggtggtaccttctttcgaaagttcctcagtgactcacaaaatatgttatctatattccaaaataaaaatcccaataaaaatatacccaatgatgtataacccagtcctctaagccatggataaacccatgtaacaatataaatagatcgaagtactaatgtaaagaccaacattccatacatgacctgatggaatatcggctcttttaccttaaggtaaactgtggttactattaaactgaatagaactaaggtaaaaagcagatggtagtttactgagttcttgatcttgaaacattcaaacatgcagtacacaaatatgcaacagctgtatatcattgggagttcatccaatagctgcatttcatatttcagagtcatgtggaagcaccaggatcccattcctaccactgtgagtgctaaataagaagcaatgtaccgcttttccagaccgtctctaacactctgaactgcaccgaacattggaggtataatcatgatcaggttactcactgtattcccactaggtgctgctgacagccacgttctgcaatagcctggcaccagaagctgaccaagctttaagaggtgggcactggggaagcctcagcactgtaggagccagaagctattaagccacttggactgcaagagctggcgccag

SEQ ID NO: 14303 - RNA, 4433 nt, Homo sapiens
  source 1..4433: mol_type = other RNA
gctgggattacaggcatgagccaccgcgcccggcccattatttttaaatagttagaacatagtgaataagctataattgtagacactgaaaaacaagacaaagtgatcaaactaattatagcactgacaggatgcaaaatggaagacagaggtaggtctgcaaacagccacacaggtggaaattccaattgtaaatggttctctttgaaatactcagttttacataaatgcttatccagcagcacgtcataaaccacagggccaaaacaatttcttgtcacgtaaacatggcgttggtagctaaaactcaaatttagcaacaaataattgttttcataggactcataagataaccttaaattgttagatgcttttagggcattggctaattcagaattggctggtattataacagaacttaatttttgcaggcatttaaagattttcatgcattatgtacctgaaggttttgtctcttaattttctttgaaccacacctcttctccttattataagaaaaaccctcttagggtaagggaagtccaaattaactgtcctgaaattttgcattatatttaaaccataatatttgatttacttctgtcaaacaaaacactactatttgggttctcatttgtagattatttaaaaacatgtttttcctgttaattatcaatgcatttactatcacaaggattaaaaagatcacttcaggtggtggggatgtttcatgaaacaccatggtggggagtaggtagtgggcaggcagagtgacaatcagcttaacctcctttcacctagctgttctttagaaaaacaaaaataaaagtcaaattgctttcagttttcaagagtgaaaatggaggcacaagaaggatattcagatgtgcaagcaaattgcttcttttacatccttatattttcttttcttttcttttttttttttttttttttttttgagacggagtctcgctctgccaccatgcccggcctcacaaagtattttctaaaatataatttgctgtagagttcacagatgagcacttttcacattaggtgatatgcaaacaaatcactattggctcagcaggaaacagactttttgtacactctagttaacatgaagttttccaataaaacaaatgacagcgggagggggtagtgaggaattcaactctgtaatgtccacctagaatccaagtaggaaaaaaataaagctattgaaataatttagtaatatcctataggtcaccagtgatttccataaaatgctgcacagatacaaagtcttgagtatgttacttagtagctaaaaagagagccttgtgtgaggcacagctgacttggaacattaaagagcctggcttccctttctgctttccattctcccaacagaaaaaaaggtcttcaaagaattggccagtcttacagctcaccttggggtgtagatgactctccactgtggtgctaggcaattttattgaacaggtggccactggtggtgatggctgaaccactcattaaacaaattgctctaaatggcctcagtatcaaggtgtgctttctgtacccttaatctgactttaatcctgcagaacctcagtcttaccatgtttaacagcattgccatgtacgatatgcctttatcctacactgtatatatactctttatgcagaagtatatctaactgaaaagtataaaaatataatggtggaaaacaaatgaattaaaaaatgtatcacggccgatagcccaggtaactgcaggtgaaatgtagccagaagtcagaatcttggggcaaaatcaagtatagtcttatgggctgtgccttcaaatggtttagttttataccctcttaaggcagaatcaaagttctcttaatgttttggcaagtgtttttcttcctggaggttcataaaaataggtggaagaatcagtctaatggcttgttggcatgctaagggaaggatgtcaagttgacatccttggatacttggttaaaaactaaggctagtaggtgaagaaaaacaacagaatagtttttggttttaaatttgtacaaaggctacttattgaatactggaaaaaatgacaacagtgttttaccatctttgcataagaaaaaaatgattttccttttgaaactgtagctcaggatttaatcctgagtcacgtcatcatgtggtaaaaacaatctggattttacaataatttatataaagcaaaaaaagtcataaaaatgctaaatgatgcagagctacaaatatgatgaaacatgagcagaggggtcaaatcagatttttactccaggcaggtgttaagtttgtgaaaagtgatgcaatttgttatacattcaaatgcaaattagaactagctgccttacgatgagatttcactgtcatttttttagcaccctaatttttgtcggttctgtaggtttcaagtagcagaaacttacatctatttccttcagaaaattaaggagcagatattttaatatgctttatgtaaataggattctgataattttagctttagttaatgcaacacacttccctgggcacaaccatgacctctctgagaactggaaaatactgcataattttaaaaatcagagtgtaatgacattccctgacaacttcaaataagttatgtgaggaggatgaactatgggtagtctagaccaccagtcatatttgtctagccgtagaaacagtgacaacttaaagatctgcaaagatcagagcagagctggctgaaggtgcagcattctatacatgtcctcatggagcttcagaaaggttataagatgacccactcattctggttggctgtggccatagacagacaccataaatcctgggatgtggtcaagtactgaactgggggcaggtctgagcttgcttatgatcctccgactagccctggaacagatagtgaagaactacacagaatcccacagctagctctctctctttctctctctttttttacctttgagaaccatccatgagattaatacaatattaatcaaatctgacacagctgagtgctggctcacagctaactatctggatatggggttttgttggctcttagctgactgcattatttaatcaaatattaagaaaggtataattcacatgcaacccttggcaaaaagaaaagaaggttaatttcttataaccagcacaaactgttaacctgttaagaaaagcccaactgtttctgcatttgaggcatacacacacatcatctctgtttctttataaactggagcgtgaaaggaggagggggacaaataagataaagccatgagctaaacacccagcaggccctactccttattctctgtgtgggtggcagcattagtcagaaagtcactcctctgctgtgatggtcatgacatatttgaacttgtagatctttaaggatttccttatttattctgccaggtctatggtaggtgcttgtttgttttcttggtggaatgattcatcaatgcttcctgagaggctcaaacaggatcactggccagattccaaagagaaacttcacttttggcctatatctcaggtaaagtgttcttgtatacaaactgaaaaggatgtgaagataggaaccaaggccagttaaaatatgccaccatgcatgaaattgtgtggtaatacctatgataggtggtaccttctttcgaaagttcctcagtgactcacaaaatatgttatctatattccaaaataaaaatcccaataaaaatatacccaatgatgtataacccagtcctctaagccatggataaacccatgtaacaatataaatagatcgaagtactaatgtaaagaccaacattccatacatgacctgatggaatatcggctcttttaccttaaggtaaactgtggttactattaaactgaatagaactaaggtaaaaagcagatggtagtttactgagttcttgatcttgaaacattcaaacatgcagtacacaaatatgcaacagctgtatatcattgggagttcatccaatagctgcttatttctttacttcacttagtcagtttggatcctcagacttgaagtaaaaaactccagagattacaaatcccatcttttagccatagttatgtgctcttttctcaaatctgaagtacttctgtgagtgctaaataagaagcaatgtaccgcttttccagaccgtctctaacactctgaactgcaccgaacattggaggtataatcatgatcaggttactcactgtattccagaactcggcgatgtaccaggtcacggagtagttctcctcgcaccagtccagcgtggaggtcgtggggccccagtagccctctcggtccgcggccggagccatcacgccgccgccgccgccgcccaggcgctccgctcactgtgccgggttaggctggcgac

SEQ ID NO: 14304 - RNA, 4309 nt, Homo sapiens
  source 1..4309: mol_type = other RNA
gctgggattacaggcatgagccaccgcgcccggcccattatttttaaatagttagaacatagtgaataagctataattgtagacactgaaaaacaagacaaagtgatcaaactaattatagcactgacaggatgcaaaatggaagacagaggtaggtctgcaaacagccacacaggtggaaattccaattgtaaatggttctctttgaaatactcagttttacataaatgcttatccagcagcacgtcataaaccacagggccaaaacaatttcttgtcacgtaaacatggcgttggtagctaaaactcaaatttagcaacaaataattgttttcataggactcataagataaccttaaattgttagatgcttttagggcattggctaattcagaattggctggtattataacagaacttaatttttgcaggcatttaaagattttcatgcattatgtacctgaaggttttgtctcttaattttctttgaaccacacctcttctccttattataagaaaaaccctcttagggtaagggaagtccaaattaactgtcctgaaattttgcattatatttaaaccataatatttgatttacttctgtcaaacaaaacactactatttgggttctcatttgtagattatttaaaaacatgtttttcctgttaattatcaatgcatttactatcacaaggattaaaaagatcacttcaggtggtggggatgtttcatgaaacaccatggtggggagtaggtagtgggcaggcagagtgacaatcagcttaacctcctttcacctagctgttctttagaaaaacaaaaataaaagtcaaattgctttcagttttcaagagtgaaaatggaggcacaagaaggatattcagatgtgcaagcaaattgcttcttttacatccttatattttcttttcttttcttttttttttttttttttttttttgagacggagtctcgctctgccaccatgcccggcctcacaaagtattttctaaaatataatttgctgtagagttcacagatgagcacttttcacattaggtgatatgcaaacaaatcactattggctcagcaggaaacagactttttgtacactctagttaacatgaagttttccaataaaacaaatgacagcgggagggggtagtgaggaattcaactctgtaatgtccacctagaatccaagtaggaaaaaaataaagctattgaaataatttagtaatatcctataggtcaccagtgatttccataaaatgctgcacagatacaaagtcttgagtatgttacttagtagctaaaaagagagccttgtgtgaggcacagctgacttggaacattaaagagcctggcttccctttctgctttccattctcccaacagaaaaaaaggtcttcaaagaattggccagtcttacagctcaccttggggtgtagatgactctccactgtggtgctaggcaattttattgaacaggtggccactggtggtgatggctgaaccactcattaaacaaattgctctaaatggcctcagtatcaaggtgtgctttctgtacccttaatctgactttaatcctgcagaacctcagtcttaccatgtttaacagcattgccatgtacgatatgcctttatcctacactgtatatatactctttatgcagaagtatatctaactgaaaagtataaaaatataatggtggaaaacaaatgaattaaaaaatgtatcacggccgatagcccaggtaactgcaggtgaaatgtagccagaagtcagaatcttggggcaaaatcaagtatagtcttatgggctgtgccttcaaatggtttagttttataccctcttaaggcagaatcaaagttctcttaatgttttggcaagtgtttttcttcctggaggttcataaaaataggtggaagaatcagtctaatggcttgttggcatgctaagggaaggatgtcaagttgacatccttggatacttggttaaaaactaaggctagtaggtgaagaaaaacaacagaatagtttttggttttaaatttgtacaaaggctacttattgaatactggaaaaaatgacaacagtgttttaccatctttgcataagaaaaaaatgattttccttttgaaactgtagctcaggatttaatcctgagtcacgtcatcatgtggtaaaaacaatctggattttacaataatttatataaagcaaaaaaagtcataaaaatgctaaatgatgcagagctacaaatatgatgaaacatgagcagaggggtcaaatcagatttttactccaggcaggtgttaagtttgtgaaaagtgatgcaatttgttatacattcaaatgcaaattagaactagctgccttacgatgagatttcactgtcatttttttagcaccctaatttttgtcggttctgtaggtttcaagtagcagaaacttacatctatttccttcagaaaattaaggagcagatattttaatatgctttatgtaaataggattctgataattttagctttagttaatgcaacacacttccctgggcacaaccatgacctctctgagaactggaaaatactgcataattttaaaaatcagagtgtaatgacattccctgacaacttcaaataagttatgtgaggaggatgaactatgggtagtctagaccaccagtcatatttgtctagccgtagaaacagtgacaacttaaagatctgcaaagatcagagcagagctggctgaaggtgcagcattctatacatgtcctcatggagcttcagaaaggttataagatgacccactcattctggttggctgtggccatagacagacaccataaatcctgggatgtggtcaagtactgaactgggggcaggtctgagcttgcttatgatcctccgactagccctggaacagatagtgaagaactacacagaatcccacagctagctctctctctttctctctctttttttacctttgagaaccatccatgagattaatacaatattaatcaaatctgacacagctgagtgctggctcacagctaactatctggatatggggttttgttggctcttagctgactgcattatttaatcaaatattaagaaaggtataattcacatgcaacccttggcaaaaagaaaagaaggttaatttcttataaccagcacaaactgttaacctgttaagaaaagcccaactgtttctgcatttgaggcatacacacacatcatctctgtttctttataaactggagcgtgaaaggaggagggggacaaataagataaagccatgagctaaacacccagcaggccctactccttattctctgtgtgggtggcagcattagtcagaaagtcactcctctgctgtgatggtcatgacatatttgaacttgtagatctttaaggatttccttatttattctgccaggtctatggtaggtgcttgtttgttttcttggtggaatgattcatcaatgcttcctgagaggctcaaacaggatcactggccagattccaaagagaaacttcacttttggcctatatctcaggtaaagtgttcttgtatacaaactgaaaaggatgtgaagataggaaccaaggccagttaaaatatgccaccatgcatgaaattgtgtggtaatacctatgataggtggtaccttctttcgaaagttcctcagtgactcacaaaatatgttatctatattccaaaataaaaatcccaataaaaatatacccaatgatgtataacccagtcctctaagccatggataaacccatgtaacaatataaatagatcgaagtactaatgtaaagaccaacattccatacatgacctgatggaatatcggctcttttaccttaaggtaaactgtggttactattaaactgaatagaactaaggtaaaaagcagatggtagtttactgagttcttgatcttgaaacattcaaacatgcagtacacaaatatgcaacagctgtatatcattgggagttcatccaatagctgtgagtgctaaataagaagcaatgtaccgcttttccagaccgtctctaacactctgaactgcaccgaacattggaggtataatcatgatcaggttactcactgtattccagaactcggcgatgtaccaggtcacggagtagttctcctcgcaccagtccagcgtggaggtcgtggggccccagtagccctctcggtccgcggccggagccatcacgccgccgccgccgccgcccaggcgctccgctcactgtgccgggttaggctggcgac

SEQ ID NO: 14305 - RNA, 4915 nt, Homo sapiens
  source 1..4915: mol_type = other RNA
gctgggattacaggcatgagccaccgcgcccggcccattatttttaaatagttagaacatagtgaataagctataattgtagacactgaaaaacaagacaaagtgatcaaactaattatagcactgacaggatgcaaaatggaagacagaggtaggtctgcaaacagccacacaggtggaaattccaattgtaaatggttctctttgaaatactcagttttacataaatgcttatccagcagcacgtcataaaccacagggccaaaacaatttcttgtcacgtaaacatggcgttggtagctaaaactcaaatttagcaacaaataattgttttcataggactcataagataaccttaaattgttagatgcttttagggcattggctaattcagaattggctggtattataacagaacttaatttttgcaggcatttaaagattttcatgcattatgtacctgaaggttttgtctcttaattttctttgaaccacacctcttctccttattataagaaaaaccctcttagggtaagggaagtccaaattaactgtcctgaaattttgcattatatttaaaccataatatttgatttacttctgtcaaacaaaacactactatttgggttctcatttgtagattatttaaaaacatgtttttcctgttaattatcaatgcatttactatcacaaggattaaaaagatcacttcaggtggtggggatgtttcatgaaacaccatggtggggagtaggtagtgggcaggcagagtgacaatcagcttaacctcctttcacctagctgttctttagaaaaacaaaaataaaagtcaaattgctttcagttttcaagagtgaaaatggaggcacaagaaggatattcagatgtgcaagcaaattgcttcttttacatccttatattttcttttcttttcttttttttttttttttttttttttgagacggagtctcgctctgccaccatgcccggcctcacaaagtattttctaaaatataatttgctgtagagttcacagatgagcacttttcacattaggtgatatgcaaacaaatcactattggctcagcaggaaacagactttttgtacactctagttaacatgaagttttccaataaaacaaatgacagcgggagggggtagtgaggaattcaactctgtaatgtccacctagaatccaagtaggaaaaaaataaagctattgaaataatttagtaatatcctataggtcaccagtgatttccataaaatgctgcacagatacaaagtcttgagtatgttacttagtagctaaaaagagagccttgtgtgaggcacagctgacttggaacattaaagagcctggcttccctttctgctttccattctcccaacagaaaaaaaggtcttcaaagaattggccagtcttacagctcaccttggggtgtagatgactctccactgtggtgctaggcaattttattgaacaggtggccactggtggtgatggctgaaccactcattaaacaaattgctctaaatggcctcagtatcaaggtgtgctttctgtacccttaatctgactttaatcctgcagaacctcagtcttaccatgtttaacagcattgccatgtacgatatgcctttatcctacactgtatatatactctttatgcagaagtatatctaactgaaaagtataaaaatataatggtggaaaacaaatgaattaaaaaatgtatcacggccgatagcccaggtaactgcaggtgaaatgtagccagaagtcagaatcttggggcaaaatcaagtatagtcttatgggctgtgccttcaaatggtttagttttataccctcttaaggcagaatcaaagttctcttaatgttttggcaagtgtttttcttcctggaggttcataaaaataggtggaagaatcagtctaatggcttgttggcatgctaagggaaggatgtcaagttgacatccttggatacttggttaaaaactaaggctagtaggtgaagaaaaacaacagaatagtttttggttttaaatttgtacaaaggctacttattgaatactggaaaaaatgacaacagtgttttaccatctttgcataagaaaaaaatgattttccttttgaaactgtagctcaggatttaatcctgagtcacgtcatcatgtggtaaaaacaatctggattttacaataatttatataaagcaaaaaaagtcataaaaatgctaaatgatgcagagctacaaatatgatgaaacatgagcagaggggtcaaatcagatttttactccaggcaggtgttaagtttgtgaaaagtgatgcaatttgttatacattcaaatgcaaattagaactagctgccttacgatgagatttcactgtcatttttttagcaccctaatttttgtcggttctgtaggtttcaagtagcagaaacttacatctatttccttcagaaaattaaggagcagatattttaatatgctttatgtaaataggattctgataattttagctttagttaatgcaacacacttccctgggcacaaccatgacctctctgagaactggaaaatactgcataattttaaaaatcagagtgtaatgacattccctgacaacttcaaataagttatgtgaggaggatgaactatgggtagtctagaccaccagtcatatttgtctagccgtagaaacagtgacaacttaaagatctgcaaagatcagagcagagctggctgaaggtgcagcattctatacatgtcctcatggagcttcagaaaggttataagatgacccactcattctggttggctgtggccatagacagacaccataaatcctgggatgtggtcaagtactgaactgggggcaggtctgagcttgcttatgatcctccgactagccctggaacagatagtgaagaactacacagaatcccacagctagctctctctctttctctctctttttttacctttgagaaccatccatgagattaatacaatattaatcaaatctgacacagctgagtgctggctcacagctaactatctggatatggggttttgttggctcttagctgactgcattatttaatcaaatattaagaaaggtataattcacatgcaacccttggcaaaaagaaaagaaggttaatttcttataaccagcacaaactgttaacctgttaagaaaagcccaactgtttctgcatttgaggcatacacacacatcatctctgtttctttataaactggagcgtgaaaggaggagggggacaaataagataaagccatgagctaaacacccagcaggccctactccttattctctgtgtgggtggcagcattagtcagaaagtcactcctctgctgtgatggtcatgacatatttgaacttgtagatctttaaggatttccttatttattctgccaggtctatggtaggtgcttgtttgttttcttggtggaatgattcatcaatgcttcctgagaggctcaaacaggatcactggccagattccaaagagaaacttcacttttggcctatatctcaggtaaagtgttcttgtatacaaactgaaaaggatgtgaagataggaaccaaggccagttaaaatatgccaccatgcatgaaattgtgtggtaatacctatgataggtggtaccttctttcgaaagttcctgtttaacctgttcagcatgctcatttcatggaaaagagggccagaaagacagtgtcttaatgacagactagaatccagagacctaagtctaagattcaaactcctgtcaatatatgattgctgacaagatggtaaaaggaacacttgcttttttagaaaataacattaagcatatgaaagtgtatatttatatacatatatttcatatgcttattacaaatcagtcttctttattcaatgaaacagatcaggcatgtttcaaaggaatagtcaacatttgattaactatatagttctttgatgcccacacacacaaaacccaaaccctacagaggttatgaaatagtctcaggtccaaaattttaggtaatttaaacaggtattctaatagtctaactttattatactgtatatatcttttaaatgtcaacaatagtaaaaattcatttcagggcactactatttctatatgtttataaaattctctacttaataaaatgcttccaaaaatatttctgaaggaatgaaaatatatcttacctcagtgactcacaaaatatgttatctatattccaaaataaaaatcccaataaaaatatacccaatgatgtataacccagtcctctaagccatggataaacccatgtaacaatataaatagatcgaagtactaatgtaaagaccaacattccatacatgacctgatggaatatcggctcttttaccttaaggtaaactgtggttactattaaactgaatagaactaaggtaaaaagcagatggtagtttactgagttcttgatcttgaaacattcaaacatgcagtacacaaatatgcaacagctgtatatcattgggagttcatccaatagctgcatttcatatttcagagtcatgtggaagcaccaggatcccattcctaccactgtgagtgctaaataagaagcaatgtaccgcttttccagaccgtctctaacactctgaactgcaccgaacattggaggtataatcatgatcaggttactcactgtattccagaactcggcgatgtaccaggtcacggagtagttctcctcgcaccagtccagcgtggaggtcgtggggccccagtagccctctcggtccgcggccggagccatcacgccgccgccgccgccgcccaggcgctccgctcactgtgccgggttaggctggcgaccaggccggctc

SEQ ID NO: 14306 - RNA, 700 nt, Homo sapiens
  source 1..700: mol_type = other RNA
gctgggattacaggcatgagccaccgcgcccggcccctgttgcttctttctgatcctgccatctcatcactctccctctgaagaagcgaatgttacttttggtctccatcattgtggagttaggtttcaacctcctcctctccttagagttcttccatccctccaacaggataaggctagccagccccagcccggcaggctttctgtctaccatccccccgcacccgtggggatttctccagccccagcccaaggcctcgcctccatcttcatcctttcctttgcttccctaccaaacccattctcctaaacttcctcctcaaaaacctattcatttagaccctggaagagatctgggatttaattttcatgcatttcctttttaaaaaaattgatgggaaatctgaggcccaaagaaaggtagtgacttgcccaaggtcacacagagtcgttagtttgttgatggcctgggctgggagcccctttcttcagaggccccctctccacctcaggagacaagctcttgcaaatgcaggaaggtgaagcagggagtccccaagtggtctgaggagcacccaggcttccaaagggaacgggcgctggggctgggggaagggcatgtcgcacaccaaatatcccaggaggggaaactggtccccacctgtcccctggtcccctcagtcccctcatctccgccctc

SEQ ID NO: 14307 - RNA, 6948 nt, Homo sapiens
  source 1..6948: mol_type = other RNA
gctgggattacaggcatgagccaccgcgcccggcccgatttcttgattttaaaattaaaacaaaggggtagtacagccaaaataaataagaacgtaaattgccgtatttttttttctaatggtacaagaacaatttagtaaataacatcttcaacttaagataaaaagtaggatatatttataatgaaattttcaagtattatttcaaaattaaccctgtacaaatgatatattttggaaattccaatatttgctagagaatattttttaaataccaaacatctttgtggttaatgctaccttaaccttaccaattaaccttctaaaagtatattacaacagaacacaaatagcttaaaacacaccatactgttttctccacaaaacagacaccagacaccgacatgagcacatctggcctggccagtgactcagaacctcatttcagaccagtacatctgcagaggaggccacgcggacccattctctctctcctaactcatataataaatattattttagattttcttagcaaactaggggacaacttacagaccccacctctcccagtcagccagtgtctgcagggtttcaggatttggggtaggaaacagaagatctcacacatgtcgtgctgattttaaataaggcatctgtctctgagacacctgggagagcacagccaccttcctcacggtgcctgcctgtctcttccggaagtcgcctctgcttgccacatgatgctggtgtaaccacaaaagatccaggacttctcgatgactgcagaagtacaggtgctcctacacacgagtacaggcgctcccacagacaatggtaaagattttcacttggggaacaggagtgtgaggtttgttaccgcctgcgacctacacctggctgactccaggggaaaccgcgggagtcgctgcagggagcccctggtctgctctcctcctcctcctccaccggcctctccctgtgcccccccaaaggtcagatcagatatggggcctcagtgtccttgtgcctcctgatggccgtcaggcctgaccaagggtccaagctgccccttcccagtggccagccacggtggaatcacacagggccagtggcctgagaggaagagaccagcaggaaggaaagatcctcagcaacaaagtaaaaccagaacaacagaggacctttctgtgtaagaatatttggctttagaaggtaaataaaataattatatttcttagaattttctgactatccctaaatcctgcaggtaaattattcccaacaaattttcaaaaggcaatcaataataagtaggttcttcttcaataacatgagcatatgcttcttaaagactgggtgacaggccgggcgcaggggctcacgcctgtaatcccagcactttgggaggctgagatgggcagatcacttgaggtcaggagatcgagaccatcctggccaacatggtgaaaccccattgctactaaaaatacaaacattagcctggcatagtggcgcacgcctgtaatcccagctactcgagaggctgaggcaggagaatcgcatgaacctgggaggcggagcttgcagtgagcggagagtgtgccactgcactccagcctgggcaacaaagcgagactctgtctcaaaaaaaaaaaaaaaaaaaaaacaaagattggattatgatattcagtatctatgtacacatcctatggtgggatggctatccaaaaaaacaagtaaaaagccaaaggtacagataaaatttcatttctgcggaaaagtaaagctcttactgaatggaacagggaagtgagaaactgcagccggcctggccaggcgcggtgccgcagaccctgtcacacagctgctcccagttacgcagcctctccctgtcacccgcagagagcagcatcggtggccgctcagaagccacgacctacaagtaacccttcagacacgttcaaagctcctcgccgagagcctatcaggcttttaagagttggtcattccatgtgaaaagctaattgtgatcttcgaatgtttttctagtccttggctctcattctgctatatattttacttcttgttaaaggcaaaacaaaacttaaatttcatgtcttagaaaaacatcgaccacacaatcaaataaataacattgataagagccttctggggcagcggcgcacggaggcgagtccacagcagtcactctcccggcccttctttggaagccctgctctgactgtgtctctgtgggtcgccgcgtgggccggcgtgaccccccgggggcacagggctggcagtggctggctccagcggcgtccacgaggacagagactcgtgcaccgtcagggcgtgctcctccatctggcgctgcaggctgtccatctcctgcttgagctgctggaggcagctgttcaggttcttgaggggctccttgctcacggcgggcggtggtctcagcagctcctccagcagcgaggcgggaactgggcagtccgggatcttgatgggcgtggcagggttggaagagctggcctcgcctttcggctcctttctcgtcttggccgcgccgcggcgtaggtccagcttgagctgctggttctgctggagcagggtcttcatgttgttcttcagctccgacacttttgcctggagcataaatttatccttctgggtcatggacaggtcttcctgggccatctccaactcagacttgacgttctgcagcagctgctgtagcccttccagttccttcctgccctgctgctccgtcaagtccagctgctgcttcaaggactggatttctctttctttctgatccacctcccatttgagattttccatctcttggtttcccacgggctgtttgctgagctgctcgtccagctgcttctgcaggagctggagctgtgcccgggcctcggccagctctgcttggaactgtgctatctcctgggaatgtttcccctcccgaatctgaaggtcgtcggcctcggcctgcagcttctgcaccaggtgttccttggcctgcagctccttcttcacctcactcagctccaaggaggccgccttgaagtggcggcggttatgcccggcttccaccttggcagcagccacctgctccttgaggctgttcaccttctccttctccttctctagtgaggcctgcagggcctggacaagatgcttcatctggcgatcctcctcttctttgcgctgcaaaactgcctgcacctgaaggttcaactggactaggtctgcctccctcttggccaaagctgtttctaggatgctgttgtgttcccgcagagctgcgttggactgaccgaggcccgtaagcttccctttctcgtgctctaattcaagagccaacttcttgtttgactcctcaaggcgttttatcttcttcctaaagcctctggattcttgaagctcgtcctccagctccagcaccttctcccgggactcctccagctcctggctggtcagcgctatgacctcctgcagttccttttccagcagcgtcttgctatgactgacagcctgcagctccgcctccagggcctggatcctttcatgtagagccaggctgctgtcactgctgccaccctgggctcggagctggcccagctccgcgtccgcagcctccttggccgcgagggcctcctgcaggcggcggctgaggatgcccacggcgttctcgtaggccttatgtttggtcttcatctccttctgggcgctggtcaagtctgagcccagccgcctcatcttctgcttctgttccgtgatggccttccgggcctcttgctgcaactcttcgatttgtttcttcagcgcctcattggcctctgtgaccgcgaccatctgctccttatcgaactgcaacgactgcaagtgtgtttccatctcgtctcgctccttctgcgccgactggagatgcccttcaaggtccgccatgtgctgacggacctgggccacctctctgtgcaggcgcgagagctccgcctcggcagtccgcttctccccgtgcacttgcatcagctcctgccgcagctccttcagctccgagtccagcctcttcctggtggctttcagctcactgatgagctggtctttggaggtggcgtcgcgccggtaggcctccaccatcaccttttgttggagaaactgttcctttattttttgcatttgctttttcagagcagcagtctcctgctgcaggtgttccacctggccggatttgatagctaattcttctcttaacttctctaaagtttccgacgtttcctcggtaccttcttccaagcgtcttgctcctctgtcaagctcctccttgccactcttggccgcctgcaaagccgcctccaagatgatcttctcgttctgcaggaggcagatcgtgtcctccctggaggcggcctcgccctgcagctcccccagcctggcctgcagctcatcgtagtgtgtctgcagggcatcgagggactgctccctgctctgcagagcctcctgagtcaaggtgagctgtttcatcaggtccaggtgctcctgctgcaaagcctcaagctgctggtctcgctggagtaaagtcaacttcacctgctccagctgctgctccagggatgccgccgagtccgccatcctctgcagccgctccctctcaccttcaaactcttccagcctcctctgaaggtcctcctccaccatcgtctttgcctcctgaatctgcatgaaggctgcttcctgatccaacatgtcagcctcaatgccctgcagctgtgccgcgatgcgccccttctccttcatggacctgtgctgagtttccgtcagctgctgggacagggacacattctcgagtttcaggtgctccaggagacctgcctgggtcatctgtccaacctggatgtgggccatctcaccctgcagcctgacgcgggcctcctgtgccagggcgagctgctgctggtaccactgccggacactctgcagggacgagatctccgcctgcgacgccttcagcttgctggtcagcgtcgtccgctccagctgcacctgctgaagctggctctgcaaggctgtcatctgctgtcgcaggtcgtgcactgtgttgtccttgctgagcatgctcctctgcatgtcctctaccttggccataagcctctggtactgctcctcggccacctgcaagtcgttgttggacgacgccaggctggcattttttgcctccagcatgttctgcaggtcagtcatggctcgctccaggtcccagcacgactgcttcagggtgtccacctccgagctcagcgaatcctgccgctgctggctgctgtggctgcactccacctgcgcctgcagcttcgtgctgagggcggccagctgggcctgcagctcagccttctctttaagtgcctgactcgcctccagtgacaaggcttccagctgtccttcgagtcgcattttctctttgagcacctgcagcatctcctcctgtgtttctgctgcagagctctccaaggacacgctgctgcagatgctgtctctccgactccgcacctccccgttgacctcctgcccctggtcttggtgctcagcggctgcggcctggaggacgtccttaatggaggggaactggcccagggtatccgcaggaatctcctggccgttgaccatatagggggtgtcctgcgtgcccactgtcttcgacagaatgccataggtccctcgggtggaggcgctgctgtacgatgagctgtcgctgtcatttccatccacctcagacacgctgtctccagccagggaggtgttctccagacggtcgtcagtgtcgggggacaggctgatctcagacacaacggacgccgcactgcttctgttctgcttcagggaacccttggtagaatcgggagccgggacatttcccccagaattccccgcatttgaatcttcagttctgtaatcggccagagaccggattttgcttgatttggaagtttttttctccctaggatgtgccggaagccccaggctgcccaccttaggcccccgagggacactggtgcgcaggaaggaatattcttttgtcatagccagggtactggcccttggtaagttttctgggtttaacatgagctcaggatcaagcgtgctaaaaagtctcgttttggttgcaggttgactggacctctcctgctggcgcttcaccctgtactgtttgagctgctcttccagccacttccgagcctgaagtcggacctgctcctccttctccaggggcaggggagaatctgtagagcacagttgcgtttcttgcataggaagactgagtctgagagactgcaaagcttcttttctaacactgccctcagcactagttccctgagacttccttaggttgtcatggaaaccagccacacctggagaggcatcagggcccactgggcttgtggtgggatcgagagacgacggagggtctgggaagggtggcgttggcccgttctgacagaggcctccctggccaggtccatccgggctttccccttccgtggatgctctgtttacctcggcacactggactttgtcctgctggtcaggtggcaccagtgggcccgggggcttcagtggggcctcggggagagacgaggggccactgtgggatctgtcctcctggaggccatcttgctcggccgacgcgccgtccatggtcaggacgacaccagctgagctgacgctgaggggctacaagtgaaccttggacaagcttggcttctgccatcagcaacagccaagagctcctgggaggggccctactgtgtctcccattttcaggagaagatctgatgactcacaaatgacttgatgtcaaaccagctaatatcatgatacccgtgacaacgcccggccccactcgctctggccacctggaatgaagacaagtcggccagcgac

SEQ ID NO: 14308 - RNA, 6988 nt, Homo sapiens
  source 1..6988: mol_type = other RNA
gctgggattacaggcatgagccaccgcgcccggcccgatttcttgattttaaaattaaaacaaaggggtagtacagccaaaataaataagaacgtaaattgccgtatttttttttctaatggtacaagaacaatttagtaaataacatcttcaacttaagataaaaagtaggatatatttataatgaaattttcaagtattatttcaaaattaaccctgtacaaatgatatattttggaaattccaatatttgctagagaatattttttaaataccaaacatctttgtggttaatgctaccttaaccttaccaattaaccttctaaaagtatattacaacagaacacaaatagcttaaaacacaccatactgttttctccacaaaacagacaccagacaccgacatgagcacatctggcctggccagtgactcagaacctcatttcagaccagtacatctgcagaggaggccacgcggacccattctctctctcctaactcatataataaatattattttagattttcttagcaaactaggggacaacttacagaccccacctctcccagtcagccagtgtctgcagggtttcaggatttggggtaggaaacagaagatctcacacatgtcgtgctgattttaaataaggcatctgtctctgagacacctgggagagcacagccaccttcctcacggtgcctgcctgtctcttccggaagtcgcctctgcttgccacatgatgctggtgtaaccacaaaagatccaggacttctcgatgactgcagaagtacaggtgctcctacacacgagtacaggcgctcccacagacaatggtaaagattttcacttggggaacaggagtgtgaggtttgttaccgcctgcgacctacacctggctgactccaggggaaaccgcgggagtcgctgcagggagcccctggtctgctctcctcctcctcctccaccggcctctccctgtgcccccccaaaggtcagatcagatatggggcctcagtgtccttgtgcctcctgatggccgtcaggcctgaccaagggtccaagctgccccttcccagtggccagccacggtggaatcacacagggccagtggcctgagaggaagagaccagcaggaaggaaagatcctcagcaacaaagtaaaaccagaacaacagaggacctttctgtgtaagaatatttggctttagaaggtaaataaaataattatatttcttagaattttctgactatccctaaatcctgcaggtaaattattcccaacaaattttcaaaaggcaatcaataataagtaggttcttcttcaataacatgagcatatgcttcttaaagactgggtgacaggccgggcgcaggggctcacgcctgtaatcccagcactttgggaggctgagatgggcagatcacttgaggtcaggagatcgagaccatcctggccaacatggtgaaaccccattgctactaaaaatacaaacattagcctggcatagtggcgcacgcctgtaatcccagctactcgagaggctgaggcaggagaatcgcatgaacctgggaggcggagcttgcagtgagcggagagtgtgccactgcactccagcctgggcaacaaagcgagactctgtctcaaaaaaaaaaaaaaaaaaaaaacaaagattggattatgatattcagtatctatgtacacatcctatggtgggatggctatccaaaaaaacaagtaaaaagccaaaggtacagataaaatttcatttctgcggaaaagtaaagctcttactgaatggaacagggaagtgagaaactgcagccggcctggccaggcgcggtgccgcagaccctgtcacacagctgctcccagttacgcagcctctccctgtcacccgcagagagcagcatcggtggccgctcagaagccacgacctacaagtaacccttcagacacgttcaaagctcctcgccgagagcctatcaggcttttaagagttggtcattccatgtgaaaagctaattgtgatcttcgaatgtttttctagtccttggctctcattctgctatatattttacttcttgttaaaggcaaaacaaaacttaaatttcatgtcttagaaaaacatcgaccacacaatcaaataaataacattgataagagccttctggggcagcggcgcacggaggcgagtccacagcagtcactctcccggcccttctttggaagccctgctctgactgtgtctctgtgggtcgccgcgtgggccggcgtgaccccccgggggcacagggctggcagtggctggctccagcggcgtccacgaggacagagactcgtgcaccgtcagggcgtgctcctccatctggcgctgcaggctgtccatctcctgcttgagctgctggaggcagctgttcaggttcttgaggggctccttgctcacggcgggcggtggtctcagcagctcctccagcagcgaggcgggaactgggcagtccgggatcttgatgggcgtggcagggttggaagagctggcctcgcctttcggctcctttctcgtcttggccgcgccgcggcgtaggtccagcttgagctgctggttctgctggagcagggtcttcatgttgttcttcagctccgacacttttgcctggagcataaatttatccttctgggtcatggacaggtcttcctgggccatctccaactcagacttgacgttctgcagcagctgctgtagcccttccagttccttcctgccctgctgctccgtcaagtccagctgctgcttcaaggactggatttctctttctttctgatccacctcccatttgagattttccatctcttggtttcccacgggctgtttgctgagctgctcgtccagctgcttctgcaggagctggagctgtgcccgggcctcggccagctctgcttggaactgtgctatctcctgggaatgtttcccctcccgaatctgaaggtcgtcggcctcggcctgcagcttctgcaccaggtgttccttggcctgcagctccttcttcacctcactcagctccaaggaggccgccttgaagtggcggcggttatgcccggcttccaccttggcagcagccacctgctccttgaggctgttcaccttctccttctccttctctagtgaggcctgcagggcctggacaagatgcttcatctggcgatcctcctcttctttgcgctgcaaaactgcctgcacctgaaggttcaactggactaggtctgcctccctcttggccaaagctgtttctaggatgctgttgtgttcccgcagagctgcgttggactgaccgaggcccgtaagcttccctttctcgtgctctaattcaagagccaacttcttgtttgactcctcaaggcgttttatcttcttcctaaagcctctggattcttgaagctcgtcctccagctccagcaccttctcccgggactcctccagctcctggctggtcagcgctatgacctcctgcagttccttttccagcagcgtcttgctatgactgacagcctgcagctccgcctccagggcctggatcctttcatgtagagccaggctgctgtcactgctgccaccctgggctcggagctggcccagctccgcgtccgcagcctccttggccgcgagggcctcctgcaggcggcggctgaggatgcccacggcgttctcgtaggccttatgtttggtcttcatctccttctgggcgctggtcaagtctgagcccagccgcctcatcttctgcttctgttccgtgatggccttccgggcctcttgctgcaactcttcgatttgtttcttcagcgcctcattggcctctgtgaccgcgaccatctgctccttatcgaactgcaacgactgcaagtgtgtttccatctcgtctcgctccttctgcgccgactggagatgcccttcaaggtccgccatgtgctgacggacctgggccacctctctgtgcaggcgcgagagctccgcctcggcagtccgcttctccccgtgcacttgcatcagctcctgccgcagctccttcagctccgagtccagcctcttcctggtggctttcagctcactgatgagctggtctttggaggtggcgtcgcgccggtaggcctccaccatcaccttttgttggagaaactgttcctttattttttgcatttgctttttcagagcagcagtctcctgctgcaggtgttccacctggccggatttgatagctaattcttctcttaacttctctaaagtttccgacgtttcctcggtaccttcttccaagcgtcttgctcctctgtcaagctcctccttgccactcttggccgcctgcaaagccgcctccaagatgatcttctcgttctgcaggaggcagatcgtgtcctccctggaggcggcctcgccctgcagctcccccagcctggcctgcagctcatcgtagtgtgtctgcagggcatcgagggactgctccctgctctgcagagcctcctgagtcaaggtgagctgtttcatcaggtccaggtgctcctgctgcaaagcctcaagctgctggtctcgctggagtaaagtcaacttcacctgctccagctgctgctccagggatgccgccgagtccgccatcctctgcagccgctccctctcaccttcaaactcttccagcctcctctgaaggtcctcctccaccatcgtctttgcctcctgaatctgcatgaaggctgcttcctgatccaacatgtcagcctcaatgccctgcagctgtgccgcgatgcgccccttctccttcatggacctgtgctgagtttccgtcagctgctgggacagggacacattctcgagtttcaggtgctccaggagacctgcctgggtcatctgtccaacctggatgtgggccatctcaccctgcagcctgacgcgggcctcctgtgccagggcgagctgctgctggtaccactgccggacactctgcagggacgagatctccgcctgcgacgccttcagcttgctggtcagcgtcgtccgctccagctgcacctgctgaagctggctctgcaaggctgtcatctgctgtcgcaggtcgtgcactgtgttgtccttgctgagcatgctcctctgcatgtcctctaccttggccataagcctctggtactgctcctcggccacctgcaagtcgttgttggacgacgccaggctggcattttttgcctccagcatgttctgcaggtcagtcatggctcgctccaggtcccagcacgactgcttcagggtgtccacctccgagctcagcgaatcctgccgctgctggctgctgtggctgcactccacctgcgcctgcagcttcgtgctgagggcggccagctgggcctgcagctcagccttctctttaagtgcctgactcgcctccagtgacaaggcttccagctgtccttcgagtcgcattttctctttgagcacctgcagcatctcctcctgtgtttctgctgcagagctctccaaggacacgctgctgcagatgctgtctctccgactccgcacctccccgttgacctcctgcccctggtcttggtgctcagcggctgcggcctggaggacgtccttaatggaggggaactggcccagggtatccgcaggaatctcctggccgttgaccatatagggggtgtcctgcgtgcccactgtcttcgacagaatgccataggtccctcgggtggaggcgctgctgtacgatgagctgtcgctgtcatttccatccacctcagacacgctgtctccagccagggaggtgttctccagacggtcgtcagtgtcgggggacaggctgatctcagacacaacggacgccgcactgcttctgttctgcttcagggaacccttggtagaatcgggagccgggacatttcccccagaattccccgcatttgaatcttcagttctgtaatcggccagagaccggattttgcttgatttggaagtttttttctccctaggatgtgccggaagccccaggctgcccaccttaggcccccgagggacactggtgcgcaggaaggaatattcttttgtcatagccagggtactggcccttggtaagttttctgggtttaacatgagctcaggatcaagcgtgctaaaaagtctcgttttggttgcaggttgactggacctctcctgctggcgcttcaccctgtactgtttgagctgctcttccagccacttccgagcctgaagtcggacctgctcctccttctccaggggcaggggagaatctgtagagcacagttgcgtttcttgcataggaagactgagtctgagagactgcaaagcttcttttctaacactgccctcagcactagttccctgagacttccttaggttgtcatggaaaccagccacacctggagaggcatcagggcccactgggcttgtggtgggatcgagagacgacggagggtctgggaagggtggcgttggcccgttctgacagaggcctccctggccaggtccatccgggctttccccttccgtggatgctctgtttacctcggcacactggactttgtcctgctggtcaggtggcaccagtgggcccgggggcttcagtggggcctcggggagagacgaggggccactgtgggatctgtcctcctggaggccatcttgctcggccgacgcgccgtccatggtcaggacgacaccagctgagctgacgctgaggggctacaagtgaaccttggacaagcttggcttctgccatcagcaacagccaagagctcctgggaggggccctactgtgtctcccattttcaggagaagatctgatgactcacaaatgacttgatgtcaaaccagctaatatcatgataccctgctgctctggcagccccggaggccgcccggcccggatgctccggcggagacgtggccgtgagaggggcggggcgagcggtgcatcggcctcgggtccccg

SEQ ID NO: 14309 - RNA, 6998 nt, Homo sapiens
  source 1..6998: mol_type = other RNA
gctgggattacaggcatgagccaccgcgcccggcccgatttcttgattttaaaattaaaacaaaggggtagtacagccaaaataaataagaacgtaaattgccgtatttttttttctaatggtacaagaacaatttagtaaataacatcttcaacttaagataaaaagtaggatatatttataatgaaattttcaagtattatttcaaaattaaccctgtacaaatgatatattttggaaattccaatatttgctagagaatattttttaaataccaaacatctttgtggttaatgctaccttaaccttaccaattaaccttctaaaagtatattacaacagaacacaaatagcttaaaacacaccatactgttttctccacaaaacagacaccagacaccgacatgagcacatctggcctggccagtgactcagaacctcatttcagaccagtacatctgcagaggaggccacgcggacccattctctctctcctaactcatataataaatattattttagattttcttagcaaactaggggacaacttacagaccccacctctcccagtcagccagtgtctgcagggtttcaggatttggggtaggaaacagaagatctcacacatgtcgtgctgattttaaataaggcatctgtctctgagacacctgggagagcacagccaccttcctcacggtgcctgcctgtctcttccggaagtcgcctctgcttgccacatgatgctggtgtaaccacaaaagatccaggacttctcgatgactgcagaagtacaggtgctcctacacacgagtacaggcgctcccacagacaatggtaaagattttcacttggggaacaggagtgtgaggtttgttaccgcctgcgacctacacctggctgactccaggggaaaccgcgggagtcgctgcagggagcccctggtctgctctcctcctcctcctccaccggcctctccctgtgcccccccaaaggtcagatcagatatggggcctcagtgtccttgtgcctcctgatggccgtcaggcctgaccaagggtccaagctgccccttcccagtggccagccacggtggaatcacacagggccagtggcctgagaggaagagaccagcaggaaggaaagatcctcagcaacaaagtaaaaccagaacaacagaggacctttctgtgtaagaatatttggctttagaaggtaaataaaataattatatttcttagaattttctgactatccctaaatcctgcaggtaaattattcccaacaaattttcaaaaggcaatcaataataagtaggttcttcttcaataacatgagcatatgcttcttaaagactgggtgacaggccgggcgcaggggctcacgcctgtaatcccagcactttgggaggctgagatgggcagatcacttgaggtcaggagatcgagaccatcctggccaacatggtgaaaccccattgctactaaaaatacaaacattagcctggcatagtggcgcacgcctgtaatcccagctactcgagaggctgaggcaggagaatcgcatgaacctgggaggcggagcttgcagtgagcggagagtgtgccactgcactccagcctgggcaacaaagcgagactctgtctcaaaaaaaaaaaaaaaaaaaaaacaaagattggattatgatattcagtatctatgtacacatcctatggtgggatggctatccaaaaaaacaagtaaaaagccaaaggtacagataaaatttcatttctgcggaaaagtaaagctcttactgaatggaacagggaagtgagaaactgcagccggcctggccaggcgcggtgccgcagaccctgtcacacagctgctcccagttacgcagcctctccctgtcacccgcagagagcagcatcggtggccgctcagaagccacgacctacaagtaacccttcagacacgttcaaagctcctcgccgagagcctatcaggcttttaagagttggtcattccatgtgaaaagctaattgtgatcttcgaatgtttttctagtccttggctctcattctgctatatattttacttcttgttaaaggcaaaacaaaacttaaatttcatgtcttagaaaaacatcgaccacacaatcaaataaataacattgataagagccttctggggcagcggcgcacggaggcgagtccacagcagtcactctcccggcccttctttggaagccctgctctgactgtgtctctgtgggtcgccgcgtgggccggcgtgaccccccgggggcacagggctggcagtggctggctccagcggcgtccacgaggacagagactcgtgcaccgtcagggcgtgctcctccatctggcgctgcaggctgtccatctcctgcttgagctgctggaggcagctgttcaggttcttgaggggctccttgctcacggcgggcggtggtctcagcagctcctccagcagcgaggcgggaactgggcagtccgggatcttgatgggcgtggcagggttggaagagctggcctcgcctttcggctcctttctcgtcttggccgcgccgcggcgtaggtccagcttgagctgctggttctgctggagcagggtcttcatgttgttcttcagctccgacacttttgcctggagcataaatttatccttctgggtcatggacaggtcttcctgggccatctccaactcagacttgacgttctgcagcagctgctgtagcccttccagttccttcctgccctgctgctccgtcaagtccagctgctgcttcaaggactggatttctctttctttctgatccacctcccatttgagattttccatctcttggtttcccacgggctgtttgctgagctgctcgtccagctgcttctgcaggagctggagctgtgcccgggcctcggccagctctgcttggaactgtgctatctcctgggaatgtttcccctcccgaatctgaaggtcgtcggcctcggcctgcagcttctgcaccaggtgttccttggcctgcagctccttcttcacctcactcagctccaaggaggccgccttgaagtggcggcggttatgcccggcttccaccttggcagcagccacctgctccttgaggctgttcaccttctccttctccttctctagtgaggcctgcagggcctggacaagatgcttcatctggcgatcctcctcttctttgcgctgcaaaactgcctgcacctgaaggttcaactggactaggtctgcctccctcttggccaaagctgtttctaggatgctgttgtgttcccgcagagctgcgttggactgaccgaggcccgtaagcttccctttctcgtgctctaattcaagagccaacttcttgtttgactcctcaaggcgttttatcttcttcctaaagcctctggattcttgaagctcgtcctccagctccagcaccttctcccgggactcctccagctcctggctggtcagcgctatgacctcctgcagttccttttccagcagcgtcttgctatgactgacagcctgcagctccgcctccagggcctggatcctttcatgtagagccaggctgctgtcactgctgccaccctgggctcggagctggcccagctccgcgtccgcagcctccttggccgcgagggcctcctgcaggcggcggctgaggatgcccacggcgttctcgtaggccttatgtttggtcttcatctccttctgggcgctggtcaagtctgagcccagccgcctcatcttctgcttctgttccgtgatggccttccgggcctcttgctgcaactcttcgatttgtttcttcagcgcctcattggcctctgtgaccgcgaccatctgctccttatcgaactgcaacgactgcaagtgtgtttccatctcgtctcgctccttctgcgccgactggagatgcccttcaaggtccgccatgtgctgacggacctgggccacctctctgtgcaggcgcgagagctccgcctcggcagtccgcttctccccgtgcacttgcatcagctcctgccgcagctccttcagctccgagtccagcctcttcctggtggctttcagctcactgatgagctggtctttggaggtggcgtcgcgccggtaggcctccaccatcaccttttgttggagaaactgttcctttattttttgcatttgctttttcagagcagcagtctcctgctgcaggtgttccacctggccggatttgatagctaattcttctcttaacttctctaaagtttccgacgtttcctcggtaccttcttccaagcgtcttgctcctctgtcaagctcctccttgccactcttggccgcctgcaaagccgcctccaagatgatcttctcgttctgcaggaggcagatcgtgtcctccctggaggcggcctcgccctgcagctcccccagcctggcctgcagctcatcgtagtgtgtctgcagggcatcgagggactgctccctgctctgcagagcctcctgagtcaaggtgagctgtttcatcaggtccaggtgctcctgctgcaaagcctcaagctgctggtctcgctggagtaaagtcaacttcacctgctccagctgctgctccagggatgccgccgagtccgccatcctctgcagccgctccctctcaccttcaaactcttccagcctcctctgaaggtcctcctccaccatcgtctttgcctcctgaatctgcatgaaggctgcttcctgatccaacatgtcagcctcaatgccctgcagctgtgccgcgatgcgccccttctccttcatggacctgtgctgagtttccgtcagctgctgggacagggacacattctcgagtttcaggtgctccaggagacctgcctgggtcatctgtccaacctggatgtgggccatctcaccctgcagcctgacgcgggcctcctgtgccagggcgagctgctgctggtaccactgccggacactctgcagggacgagatctccgcctgcgacgccttcagcttgctggtcagcgtcgtccgctccagctgcacctgctgaagctggctctgcaaggctgtcatctgctgtcgcaggtcgtgcactgtgttgtccttgctgagcatgctcctctgcatgtcctctaccttggccataagcctctggtactgctcctcggccacctgcaagtcgttgttggacgacgccaggctggcattttttgcctccagcatgttctgcaggtcagtcatggctcgctccaggtcccagcacgactgcttcagggtgtccacctccgagctcagcgaatcctgccgctgctggctgctgtggctgcactccacctgcgcctgcagcttcgtgctgagggcggccagctgggcctgcagctcagccttctctttaagtgcctgactcgcctccagtgacaaggcttccagctgtccttcgagtcgcattttctctttgagcacctgcagcatctcctcctgtgtttctgctgcagagctctccaaggacacgctgctgcagatgctgtctctccgactccgcacctccccgttgacctcctgcccctggtcttggtgctcagcggctgcggcctggaggacgtccttaatggaggggaactggcccagggtatccgcaggaatctcctggccgttgaccatatagggggtgtcctgcgtgcccactgtcttcgacagaatgccataggtccctcgggtggaggcgctgctgtacgatgagctgtcgctgtcatttccatccacctcagacacgctgtctccagccagggaggtgttctccagacggtcgtcagtgtcgggggacaggctgatctcagacacaacggacgccgcactgcttctgttctgcttcagggaacccttggtagaatcgggagccgggacatttcccccagaattccccgcatttgaatcttcagttctgtaatcggccagagaccggattttgcttgatttggaagtttttttctccctaggatgtgccggaagccccaggctgcccaccttaggcccccgagggacactggtgcgcaggaaggaatattcttttgtcatagccagggtactggcccttggtaagttttctgggtttaacatgagctcaggatcaagcgtgctaaaaagtctcgttttggttgcaggttgactggacctctcctgctggcgcttcaccctgtactgtttgagctgctcttccagccacttccgagcctgaagtcggacctgctcctccttctccaggggcaggggagaatctgtagagcacagttgcgtttcttgcataggaagactgagtctgagagactgcaaagcttcttttctaacactgccctcagcactagttccctgagacttccttaggttgtcatggaaaccagccacacctggagaggcatcagggcccactgggcttgtggtgggatcgagagacgacggagggtctgggaagggtggcgttggcccgttctgacagaggcctccctggccaggtccatccgggctttccccttccgtggatgctctgtttacctcggcacactggactttgtcctgctggtcaggtggcaccagtgggcccgggggcttcagtggggcctcggggagagacgaggggccactgtgggatctgtcctcctggaggccatcttgctcggccgacgcgccgtccatggtcaggacgacaccagctgagctgacgctgaggggctacaagtgaaccttggacaagcttggcttctgccatcagcaacagccaagagctcctgggaggggccctactgtgtctcccattttcaggagaagatctgatgactcacaaatgacttgatgtcaaaccagctaatatcatgatacctccgactgtgatgaggccgccttcagaaagtgaccttaagagtttgcggacctttccctagtagaaacgcaacttccggaactgcaggaccaactctttcaggaagctgaac

SEQ ID NO: 14310 - RNA, 7751 nt, Homo sapiens
  source 1..7751: mol_type = other RNA
gctgggattacaggcatgagccaccgcgcccggcccgatttcttgattttaaaattaaaacaaaggggtagtacagccaaaataaataagaacgtaaattgccgtatttttttttctaatggtacaagaacaatttagtaaataacatcttcaacttaagataaaaagtaggatatatttataatgaaattttcaagtattatttcaaaattaaccctgtacaaatgatatattttggaaattccaatatttgctagagaatattttttaaataccaaacatctttgtggttaatgctaccttaaccttaccaattaaccttctaaaagtatattacaacagaacacaaatagcttaaaacacaccatactgttttctccacaaaacagacaccagacaccgacatgagcacatctggcctggccagtgactcagaacctcatttcagaccagtacatctgcagaggaggccacgcggacccattctctctctcctaactcatataataaatattattttagattttcttagcaaactaggggacaacttacagaccccacctctcccagtcagccagtgtctgcagggtttcaggatttggggtaggaaacagaagatctcacacatgtcgtgctgattttaaataaggcatctgtctctgagacacctgggagagcacagccaccttcctcacggtgcctgcctgtctcttccggaagtcgcctctgcttgccacatgatgctggtgtaaccacaaaagatccaggacttctcgatgactgcagaagtacaggtgctcctacacacgagtacaggcgctcccacagacaatggtaaagattttcacttggggaacaggagtgtgaggtttgttaccgcctgcgacctacacctggctgactccaggggaaaccgcgggagtcgctgcagggagcccctggtctgctctcctcctcctcctccaccggcctctccctgtgcccccccaaaggtcagatcagatatggggcctcagtgtccttgtgcctcctgatggccgtcaggcctgaccaagggtccaagctgccccttcccagtggccagccacggtggaatcacacagggccagtggcctgagaggaagagaccagcaggaaggaaagatcctcagcaacaaagtaaaaccagaacaacagaggacctttctgtgtaagaatatttggctttagaaggtaaataaaataattatatttcttagaattttctgactatccctaaatcctgcaggtaaattattcccaacaaattttcaaaaggcaatcaataataagtaggttcttcttcaataacatgagcatatgcttcttaaagactgggtgacaggccgggcgcaggggctcacgcctgtaatcccagcactttgggaggctgagatgggcagatcacttgaggtcaggagatcgagaccatcctggccaacatggtgaaaccccattgctactaaaaatacaaacattagcctggcatagtggcgcacgcctgtaatcccagctactcgagaggctgaggcaggagaatcgcatgaacctgggaggcggagcttgcagtgagcggagagtgtgccactgcactccagcctgggcaacaaagcgagactctgtctcaaaaaaaaaaaaaaaaaaaaaacaaagattggattatgatattcagtatctatgtacacatcctatggtgggatggctatccaaaaaaacaagtaaaaagccaaaggtacagataaaatttcatttctgcggaaaagtaaagctcttactgaatggaacagggaagtgagaaactgcagccggcctggccaggcgcggtgccgcagaccctgtcacacagctgctcccagttacgcagcctctccctgtcacccgcagagagcagcatcggtggccgctcagaagccacgacctacaagtaacccttcagacacgttcaaagctcctcgccgagagcctatcaggcttttaagagttggtcattccatgtgaaaagctaattgtgatcttcgaatgtttttctagtccttggctctcattctgctatatattttacttcttgttaaaggcaaaacaaaacttaaatttcatgtcttagaaaaacatcgaccacacaatcaaataaataacattgataagagccttctggggcagcggcgcacggaggcgagtccacagcagtcactctcccggcccttctttggaagccctgctctgactgtgtctctgtgggtcgccgcgtgggccggcgtgaccccccgggggcacagggctggcagtggctggctccagcggcgtccacgaggacagagactcgtgcaccgtcagggcgtgctcctccatctggcgctgcaggctgtccatctcctgcttgagctgctggaggcagctgttcaggttcttgaggggctccttgctcacggcgggcggtggtctcagcagctcctccagcagcgaggcgggaactgggcagtccgggatcttgatgggcgtggcagggttggaagagctggcctcgcctttcggctcctttctcgtcttggccgcgccgcggcgtaggtccagcttgagctgctggttctgctggagcagggtcttcatgttgttcttcagctccgacacttttgcctggagcataaatttatccttctgggtcatggacaggtcttcctgggccatctccaactcagacttgacgttctgcagcagctgctgtagcccttccagttccttcctgccctgctgctccgtcaagtccagctgctgcttcaaggactggatttctctttctttctgatccacctcccatttgagattttccatctcttggtttcccacgggctgtttgctgagctgctcgtccagctgcttctgcaggagctggagctgtgcccgggcctcggccagctctgcttggaactgtgctatctcctgggaatgtttcccctcccgaatctgaaggtcgtcggcctcggcctgcagcttctgcaccaggtgttccttggcctgcagctccttcttcacctcactcagctccaaggaggccgccttgaagtggcggcggttatgcccggcttccaccttggcagcagccacctgctccttgaggctgttcaccttctccttctccttctctagtgaggcctgcagggcctggacaagatgcttcatctggcgatcctcctcttctttgcgctgcaaaactgcctgcacctgaaggttcaactggactaggtctgcctccctcttggccaaagctgtttctaggatgctgttgtgttcccgcagagctgcgttggactgaccgaggcccgtaagcttccctttctcgtgctctaattcaagagccaacttcttgtttgactcctcaaggcgttttatcttcttcctaaagcctctggattcttgaagctcgtcctccagctccagcaccttctcccgggactcctccagctcctggctggtcagcgctatgacctcctgcagttccttttccagcagcgtcttgctatgactgacagcctgcagctccgcctccagggcctggatcctttcatgtagagccaggctgctgtcactgctgccaccctgggctcggagctggcccagctccgcgtccgcagcctccttggccgcgagggcctcctgcaggcggcggctgaggatgcccacggcgttctcgtaggccttatgtttggtcttcatctccttctgggcgctggtcaagtctgagcccagccgcctcatcttctgcttctgttccgtgatggccttccgggcctcttgctgcaactcttcgatttgtttcttcagcgcctcattggcctctgtgaccgcgaccatctgctccttatcgaactgcaacgactgcaagtgtgtttccatctcgtctcgctccttctgcgccgactggagatgcccttcaaggtccgccatgtgctgacggacctgggccacctctctgtgcaggcgcgagagctccgcctcggcagtccgcttctccccgtgcacttgcatcagctcctgccgcagctccttcagctccgagtccagcctcttcctggtggctttcagctcactgatgagctggtctttggaggtggcgtcgcgccggtaggcctccaccatcaccttttgttggagaaactgttcctttattttttgcatttgctttttcagagcagcagtctcctgctgcaggtgttccacctggccggatttgatagctaattcttctcttaacttctctaaagtttccgacgtttcctcggtaccttcttccaagcgtcttgctcctctgtcaagctcctccttgccactcttggccgcctgcaaagccgcctccaagatgatcttctcgttctgcaggaggcagatcgtgtcctccctggaggcggcctcgccctgcagctcccccagcctggcctgcagctcatcgtagtgtgtctgcagggcatcgagggactgctccctgctctgcagagcctcctgagtcaaggtgagctgtttcatcaggtccaggtgctcctgctgcaaagcctcaagctgctggtctcgctggagtaaagtcaacttcacctgctccagctgctgctccagggatgccgccgagtccgccatcctctgcagccgctccctctcaccttcaaactcttccagcctcctctgaaggtcctcctccaccatcgtctttgcctcctgaatctgcatgaaggctgcttcctgatccaacatgtcagcctcaatgccctgcagctgtgccgcgatgcgccccttctccttcatggacctgtgctgagtttccgtcagctgctgggacagggacacattctcgagtttcaggtgctccaggagacctgcctgggtcatctgtccaacctggatgtgggccatctcaccctgcagcctgacgcgggcctcctgtgccagggcgagctgctgctggtaccactgccggacactctgcagggacgagatctccgcctgcgacgccttcagcttgctggtcagcgtcgtccgctccagctgcacctgctgaagctggctctgcaaggctgtcatctgctgtcgcaggtcgtgcactgtgttgtccttgctgagcatgctcctctgcatgtcctctaccttggccataagcctctggtactgctcctcggccacctgcaagtcgttgttggacgacgccaggctggcattttttgcctccagcatgttctgcaggtcagtcatggctcgctccaggtcccagcacgactgcttcagggtgtccacctccgagctcagcgaatcctgccgctgctggctgctgtggctgcactccacctgcgcctgcagcttcgtgctgagggcggccagctgggcctgcagctcagccttctctttaagtgcctgactcgcctccagtgacaaggcttccagctgtccttcgagtcgcattttctctttgagcacctgcagcatctcctcctgtgtttctgctgcagagctctccaaggacacgctgctgcagatgctgtctctccgactccgcacctccccgttgacctcctgcccctggtcttggtgctcagcggctgcggcctggaggacgtccttaatggaggggaactggcccagggtatccgcaggaatctcctggccgttgaccatatagggggtgtcctgcgtgcccactgtcttcgacagaatgccataggtccctcgggtggaggcgctgctgtacgatgagctgtcgctgtcatttccatccacctcagacacgctgtctccagccagggaggtgttctccagacggtcgtcagtgtcgggggacaggctgatctcagacacaacggacgccgcactgcttctgttctgcttcagggaacccttggtagaatcgggagccgggacatttcccccagaattccccgcatttgaatcttcagttctgtaatcggccagagaccggattttgcttgatttggaagtttttttctccctaggatgtgccggaagccccaggctgcccaccttaggcccccgagggacactggtgcgcaggaaggaatattcttttgtcatagccagggtactggcccttggtaagttttctgggtttaacatgagctcaggatcaagcgtgctaaaaagtctcgttttggttgcaggttgactggacctctcctgctggcgcttcaccctgtactgtttgagctgctcttccagccacttccgagcctgaagtcggacctgctcctccttctccaggggcaggggagaatctgtagagcacagttgcgtttcttgcataggaagactgagtctgagagactgcaaagcttcttttctaacactgccctcagcactagttccctgagacttccttaggttgtcatggaaaccagccacacctggagaggcatcagggcccactgggcttgtggtgggatcgagagacgacggagggtctgggaagggtggcgttggcccgttctgacagaggcctccctggccaggtccatccgggctttccccttccgtggatgctctgtttacctcggcacactggactttgtcctgctggtcaggtggcaccagtgggcccgggggcttcagtggggcctcggggagagacgaggggccactgtgggatctgtcctcctggaggccatcttgctcggccgacgcgccgtccatggtcaggacgacaccagctgagctgacgctgaggggctacaagtgaaccttggacaagcttggcttctgccatcagcaacagccaagagctcctgggaggggccctactgtgtctcccattttcaggagaagatctgatgactcacaaatgacttgatgtcaaaccagctaatatcatgatacctgggaatggagaagacacccacaaaacaaggggaggagcatcagcaaaatgatggctgcttatcacaggcttgcccctttgacagatgaattacaaactggcacggaggactacacgcggtggaatgtggactcgactgcgccactgaatactggtaccctgtacatctggtcctcttgaaaatttcctagcaaaagaaaacttgcgttttgctttgtgatgtctttgcttctgccttgcgggggtggggtgattatatggaaccgaccgtgtgtgcctacgcgtgcagaccctcctggcccctcaggtaaaggaaccgacggtgtgtgcctgcgcgtgcagaccctcctggccccgcaggtaaagtgtctcgtctaccccctctgccatcactgtacctcacgtggcctccaccacagcacgtcatgtctgccattgcgtgtgtgcccattacatggcgagatccttgaagacagagactcattccccgtctgcctcccaccaccttgaacactcccaactcctaaagtgccaacacaggtttaatttgccgaattaaatcttcagttctgctgattctgctgagtacattcctctgctacaaagctaatggttccaaaacaaaatgattaagtatttgaatcctggagcatcaacactgccttttaaaatacagcaaagtctaaactagtccagctgaaacatctgtgagcttcagttccaatgagggagtccagggagttagaaactggaagagcaccttttttcagtggccgggaagatggcggacattcagactgagcgtgcctaccaaaagcagccgaccatctttcaaaacaagaagagggtcctgctgggagaaact

SEQ ID NO: 14311 - RNA, 7188 nt, Homo sapiens
  source 1..7188: mol_type = other RNA
gctgggattacaggcatgagccaccgcgcccggcccgatttcttgattttaaaattaaaacaaaggggtagtacagccaaaataaataagaacgtaaattgccgtatttttttttctaatggtacaagaacaatttagtaaataacatcttcaacttaagataaaaagtaggatatatttataatgaaattttcaagtattatttcaaaattaaccctgtacaaatgatatattttggaaattccaatatttgctagagaatattttttaaataccaaacatctttgtggttaatgctaccttaaccttaccaattaaccttctaaaagtatattacaacagaacacaaatagcttaaaacacaccatactgttttctccacaaaacagacaccagacaccgacatgagcacatctggcctggccagtgactcagaacctcatttcagaccagtacatctgcagaggaggccacgcggacccattctctctctcctaactcatataataaatattattttagattttcttagcaaactaggggacaacttacagaccccacctctcccagtcagccagtgtctgcagggtttcaggatttggggtaggaaacagaagatctcacacatgtcgtgctgattttaaataaggcatctgtctctgagacacctgggagagcacagccaccttcctcacggtgcctgcctgtctcttccggaagtcgcctctgcttgccacatgatgctggtgtaaccacaaaagatccaggacttctcgatgactgcagaagtacaggtgctcctacacacgagtacaggcgctcccacagacaatggtaaagattttcacttggggaacaggagtgtgaggtttgttaccgcctgcgacctacacctggctgactccaggggaaaccgcgggagtcgctgcagggagcccctggtctgctctcctcctcctcctccaccggcctctccctgtgcccccccaaaggtcagatcagatatggggcctcagtgtccttgtgcctcctgatggccgtcaggcctgaccaagggtccaagctgccccttcccagtggccagccacggtggaatcacacagggccagtggcctgagaggaagagaccagcaggaaggaaagatcctcagcaacaaagtaaaaccagaacaacagaggacctttctgtgtaagaatatttggctttagaaggtaaataaaataattatatttcttagaattttctgactatccctaaatcctgcaggtaaattattcccaacaaattttcaaaaggcaatcaataataagtaggttcttcttcaataacatgagcatatgcttcttaaagactgggtgacaggccgggcgcaggggctcacgcctgtaatcccagcactttgggaggctgagatgggcagatcacttgaggtcaggagatcgagaccatcctggccaacatggtgaaaccccattgctactaaaaatacaaacattagcctggcatagtggcgcacgcctgtaatcccagctactcgagaggctgaggcaggagaatcgcatgaacctgggaggcggagcttgcagtgagcggagagtgtgccactgcactccagcctgggcaacaaagcgagactctgtctcaaaaaaaaaaaaaaaaaaaaaacaaagattggattatgatattcagtatctatgtacacatcctatggtgggatggctatccaaaaaaacaagtaaaaagccaaaggtacagataaaatttcatttctgcggaaaagtaaagctcttactgaatggaacagggaagtgagaaactgcagccggcctggccaggcgcggtgccgcagaccctgtcacacagctgctcccagttacgcagcctctccctgtcacccgcagagagcagcatcggtggccgctcagaagccacgacctacaagtaacccttcagacacgttcaaagctcctcgccgagagcctatcaggcttttaagagttggtcattccatgtgaaaagctaattgtgatcttcgaatgtttttctagtccttggctctcattctgctatatattttacttcttgttaaaggcaaaacaaaacttaaatttcatgtcttagaaaaacatcgaccacacaatcaaataaataacattgataagagccttctggggcagcggcgcacggaggcgagtccacagcagtcactctcccggcccttctttggaagccctgctctgactgtgtctctgtgggtcgccgcgtgggccggcgtgaccccccgggggcacagggctggcagtggctggctccagcggcgtccacgaggacagagactcgtgcaccgtcagggcgtgctcctccatctggcgctgcaggctgtccatctcctgcttgagctgctggaggcagctgttcaggttcttgaggggctccttgctcacggcgggcggtggtctcagcagctcctccagcagcgaggcgggaactgggcagtccgggatcttgatgggcgtggcagggttggaagagctggcctcgcctttcggctcctttctcgtcttggccgcgccgcggcgtaggtccagcttgagctgctggttctgctggagcagggtcttcatgttgttcttcagctccgacacttttgcctggagcataaatttatccttctgggtcatggacaggtcttcctgggccatctccaactcagacttgacgttctgcagcagctgctgtagcccttccagttccttcctgccctgctgctccgtcaagtccagctgctgcttcaaggactggatttctctttctttctgatccacctcccatttgagattttccatctcttggtttcccacgggctgtttgctgagctgctcgtccagctgcttctgcaggagctggagctgtgcccgggcctcggccagctctgcttggaactgtgctatctcctgggaatgtttcccctcccgaatctgaaggtcgtcggcctcggcctgcagcttctgcaccaggtgttccttggcctgcagctccttcttcacctcactcagctccaaggaggccgccttgaagtggcggcggttatgcccggcttccaccttggcagcagccacctgctccttgaggctgttcaccttctccttctccttctctagtgaggcctgcagggcctggacaagatgcttcatctggcgatcctcctcttctttgcgctgcaaaactgcctgcacctgaaggttcaactggactaggtctgcctccctcttggccaaagctgtttctaggatgctgttgtgttcccgcagagctgcgttggactgaccgaggcccgtaagcttccctttctcgtgctctaattcaagagccaacttcttgtttgactcctcaaggcgttttatcttcttcctaaagcctctggattcttgaagctcgtcctccagctccagcaccttctcccgggactcctccagctcctggctggtcagcgctatgacctcctgcagttccttttccagcagcgtcttgctatgactgacagcctgcagctccgcctccagggcctggatcctttcatgtagagccaggctgctgtcactgctgccaccctgggctcggagctggcccagctccgcgtccgcagcctccttggccgcgagggcctcctgcaggcggcggctgaggatgcccacggcgttctcgtaggccttatgtttggtcttcatctccttctgggcgctggtcaagtctgagcccagccgcctcatcttctgcttctgttccgtgatggccttccgggcctcttgctgcaactcttcgatttgtttcttcagcgcctcattggcctctgtgaccgcgaccatctgctccttatcgaactgcaacgactgcaagtgtgtttccatctcgtctcgctccttctgcgccgactggagatgcccttcaaggtccgccatgtgctgacggacctgggccacctctctgtgcaggcgcgagagctccgcctcggcagtccgcttctccccgtgcacttgcatcagctcctgccgcagctccttcagctccgagtccagcctcttcctggtggctttcagctcactgatgagctggtctttggaggtggcgtcgcgccggtaggcctccaccatcaccttttgttggagaaactgttcctttattttttgcatttgctttttcagagcagcagtctcctgctgcaggtgttccacctggccggatttgatagctaattcttctcttaacttctctaaagtttccgacgtttcctcggtaccttcttccaagcgtcttgctcctctgtcaagctcctccttgccactcttggccgcctgcaaagccgcctccaagatgatcttctcgttctgcaggaggcagatcgtgtcctccctggaggcggcctcgccctgcagctcccccagcctggcctgcagctcatcgtagtgtgtctgcagggcatcgagggactgctccctgctctgcagagcctcctgagtcaaggtgagctgtttcatcaggtccaggtgctcctgctgcaaagcctcaagctgctggtctcgctggagtaaagtcaacttcacctgctccagctgctgctccagggatgccgccgagtccgccatcctctgcagccgctccctctcaccttcaaactcttccagcctcctctgaaggtcctcctccaccatcgtctttgcctcctgaatctgcatgaaggctgcttcctgatccaacatgtcagcctcaatgccctgcagctgtgccgcgatgcgccccttctccttcatggacctgtgctgagtttccgtcagctgctgggacagggacacattctcgagtttcaggtgctccaggagacctgcctgggtcatctgtccaacctggatgtgggccatctcaccctgcagcctgacgcgggcctcctgtgccagggcgagctgctgctggtaccactgccggacactctgcagggacgagatctccgcctgcgacgccttcagcttgctggtcagcgtcgtccgctccagctgcacctgctgaagctggctctgcaaggctgtcatctgctgtcgcaggtcgtgcactgtgttgtccttgctgagcatgctcctctgcatgtcctctaccttggccataagcctctggtactgctcctcggccacctgcaagtcgttgttggacgacgccaggctggcattttttgcctccagcatgttctgcaggtcagtcatggctcgctccaggtcccagcacgactgcttcagggtgtccacctccgagctcagcgaatcctgccgctgctggctgctgtggctgcactccacctgcgcctgcagcttcgtgctgagggcggccagctgggcctgcagctcagccttctctttaagtgcctgactcgcctccagtgacaaggcttccagctgtccttcgagtcgcattttctctttgagcacctgcagcatctcctcctgtgtttctgctgcagagctctccaaggacacgctgctgcagatgctgtctctccgactccgcacctccccgttgacctcctgcccctggtcttggtgctcagcggctgcggcctggaggacgtccttaatggaggggaactggcccagggtatccgcaggaatctcctggccgttgaccatatagggggtgtcctgcgtgcccactgtcttcgacagaatgccataggtccctcgggtggaggcgctgctgtacgatgagctgtcgctgtcatttccatccacctcagacacgctgtctccagccagggaggtgttctccagacggtcgtcagtgtcgggggacaggctgatctcagacacaacggacgccgcactgcttctgttctgcttcagggaacccttggtagaatcgggagccgggacatttcccccagaattccccgcatttgaatcttcagttctgtaatcggccagagaccggattttgcttgatttggaagtttttttctccctaggatgtgccggaagccccaggctgcccaccttaggcccccgagggacactggtgcgcaggaaggaatattcttttgtcatagccagggtactggcccttggtaagttttctgggtttaacatgagctcaggatcaagcgtgctaaaaagtctcgttttggttgcaggttgactggacctctcctgctggcgcttcaccctgtactgtttgagctgctcttccagccacttccgagcctgaagtcggacctgctcctccttctccaggggcaggggagaatctgtagagcacagttgcgtttcttgcataggaagactgagtctgagagactgcaaagcttcttttctaacactgccctcagcactagttccctgagacttccttaggttgtcatggaaaccagccacacctggagaggcatcagggcccactgggcttgtggtgggatcgagagacgacggagggtctgggaagggtggcgttggcccgttctgacagaggcctccctggccaggtccatccgggctttccccttccgtggatgctctgtttacctcggcacactggactttgtcctgctggtcaggtggcaccagtgggcccgggggcttcagtggggcctcggggagagacgaggggccactgtgggatctgtcctcctggaggccatcttgctcggccgacgcgccgtccatggtcaggacgacaccagctgagctgacgctgaggggctacaagtgaaccttggacaagcttggcttctgccatcagcaacagccaagagctcctgggaggggccctactgtgtctcccattttcaggagaagatctgatgactcacaaatgacttgatgtcaaaccagctaatatcatgatacttgggaaagtatgctacttcttaaggcaatcgggggaaaaaaagctcctcttcaatctgagtgatgtcagatgatttatttccttcttgccatttaaggtatactgcccgtgacaacgcccggccccactcgctctggccacctggaatgaagacaagtcggccagcgacaaagacaaacaaggaagtacacggactcctgaaaccccgacttcccacgaaccacccgacaccatgtcacgcctttcagctgcaaagggccaggctaaagcaagcactgcccgagtggtggcagtggacagct

SEQ ID NO: 14312 - RNA, 7010 nt, Homo sapiens
  source 1..7010: mol_type = other RNA
gctgggattacaggcatgagccaccgcgcccggcccgatttcttgattttaaaattaaaacaaaggggtagtacagccaaaataaataagaacgtaaattgccgtatttttttttctaatggtacaagaacaatttagtaaataacatcttcaacttaagataaaaagtaggatatatttataatgaaattttcaagtattatttcaaaattaaccctgtacaaatgatatattttggaaattccaatatttgctagagaatattttttaaataccaaacatctttgtggttaatgctaccttaaccttaccaattaaccttctaaaagtatattacaacagaacacaaatagcttaaaacacaccatactgttttctccacaaaacagacaccagacaccgacatgagcacatctggcctggccagtgactcagaacctcatttcagaccagtacatctgcagaggaggccacgcggacccattctctctctcctaactcatataataaatattattttagattttcttagcaaactaggggacaacttacagaccccacctctcccagtcagccagtgtctgcagggtttcaggatttggggtaggaaacagaagatctcacacatgtcgtgctgattttaaataaggcatctgtctctgagacacctgggagagcacagccaccttcctcacggtgcctgcctgtctcttccggaagtcgcctctgcttgccacatgatgctggtgtaaccacaaaagatccaggacttctcgatgactgcagaagtacaggtgctcctacacacgagtacaggcgctcccacagacaatggtaaagattttcacttggggaacaggagtgtgaggtttgttaccgcctgcgacctacacctggctgactccaggggaaaccgcgggagtcgctgcagggagcccctggtctgctctcctcctcctcctccaccggcctctccctgtgcccccccaaaggtcagatcagatatggggcctcagtgtccttgtgcctcctgatggccgtcaggcctgaccaagggtccaagctgccccttcccagtggccagccacggtggaatcacacagggccagtggcctgagaggaagagaccagcaggaaggaaagatcctcagcaacaaagtaaaaccagaacaacagaggacctttctgtgtaagaatatttggctttagaaggtaaataaaataattatatttcttagaattttctgactatccctaaatcctgcaggtaaattattcccaacaaattttcaaaaggcaatcaataataagtaggttcttcttcaataacatgagcatatgcttcttaaagactgggtgacaggccgggcgcaggggctcacgcctgtaatcccagcactttgggaggctgagatgggcagatcacttgaggtcaggagatcgagaccatcctggccaacatggtgaaaccccattgctactaaaaatacaaacattagcctggcatagtggcgcacgcctgtaatcccagctactcgagaggctgaggcaggagaatcgcatgaacctgggaggcggagcttgcagtgagcggagagtgtgccactgcactccagcctgggcaacaaagcgagactctgtctcaaaaaaaaaaaaaaaaaaaaaacaaagattggattatgatattcagtatctatgtacacatcctatggtgggatggctatccaaaaaaacaagtaaaaagccaaaggtacagataaaatttcatttctgcggaaaagtaaagctcttactgaatggaacagggaagtgagaaactgcagccggcctggccaggcgcggtgccgcagaccctgtcacacagctgctcccagttacgcagcctctccctgtcacccgcagagagcagcatcggtggccgctcagaagccacgacctacaagtaacccttcagacacgttcaaagctcctcgccgagagcctatcaggcttttaagagttggtcattccatgtgaaaagctaattgtgatcttcgaatgtttttctagtccttggctctcattctgctatatattttacttcttgttaaaggcaaaacaaaacttaaatttcatgtcttagaaaaacatcgaccacacaatcaaataaataacattgataagagccttctggggcagcggcgcacggaggcgagtccacagcagtcactctcccggcccttctttggaagccctgctctgactgtgtctctgtgggtcgccgcgtgggccggcgtgaccccccgggggcacagggctggcagtggctggctccagcggcgtccacgaggacagagactcgtgcaccgtcagggcgtgctcctccatctggcgctgcaggctgtccatctcctgcttgagctgctggaggcagctgttcaggttcttgaggggctccttgctcacggcgggcggtggtctcagcagctcctccagcagcgaggcgggaactgggcagtccgggatcttgatgggcgtggcagggttggaagagctggcctcgcctttcggctcctttctcgtcttggccgcgccgcggcgtaggtccagcttgagctgctggttctgctggagcagggtcttcatgttgttcttcagctccgacacttttgcctggagcataaatttatccttctgggtcatggacaggtcttcctgggccatctccaactcagacttgacgttctgcagcagctgctgtagcccttccagttccttcctgccctgctgctccgtcaagtccagctgctgcttcaaggactggatttctctttctttctgatccacctcccatttgagattttccatctcttggtttcccacgggctgtttgctgagctgctcgtccagctgcttctgcaggagctggagctgtgcccgggcctcggccagctctgcttggaactgtgctatctcctgggaatgtttcccctcccgaatctgaaggtcgtcggcctcggcctgcagcttctgcaccaggtgttccttggcctgcagctccttcttcacctcactcagctccaaggaggccgccttgaagtggcggcggttatgcccggcttccaccttggcagcagccacctgctccttgaggctgttcaccttctccttctccttctctagtgaggcctgcagggcctggacaagatgcttcatctggcgatcctcctcttctttgcgctgcaaaactgcctgcacctgaaggttcaactggactaggtctgcctccctcttggccaaagctgtttctaggatgctgttgtgttcccgcagagctgcgttggactgaccgaggcccgtaagcttccctttctcgtgctctaattcaagagccaacttcttgtttgactcctcaaggcgttttatcttcttcctaaagcctctggattcttgaagctcgtcctccagctccagcaccttctcccgggactcctccagctcctggctggtcagcgctatgacctcctgcagttccttttccagcagcgtcttgctatgactgacagcctgcagctccgcctccagggcctggatcctttcatgtagagccaggctgctgtcactgctgccaccctgggctcggagctggcccagctccgcgtccgcagcctccttggccgcgagggcctcctgcaggcggcggctgaggatgcccacggcgttctcgtaggccttatgtttggtcttcatctccttctgggcgctggtcaagtctgagcccagccgcctcatcttctgcttctgttccgtgatggccttccgggcctcttgctgcaactcttcgatttgtttcttcagcgcctcattggcctctgtgaccgcgaccatctgctccttatcgaactgcaacgactgcaagtgtgtttccatctcgtctcgctccttctgcgccgactggagatgcccttcaaggtccgccatgtgctgacggacctgggccacctctctgtgcaggcgcgagagctccgcctcggcagtccgcttctccccgtgcacttgcatcagctcctgccgcagctccttcagctccgagtccagcctcttcctggtggctttcagctcactgatgagctggtctttggaggtggcgtcgcgccggtaggcctccaccatcaccttttgttggagaaactgttcctttattttttgcatttgctttttcagagcagcagtctcctgctgcaggtgttccacctggccggatttgatagctaattcttctcttaacttctctaaagtttccgacgtttcctcggtaccttcttccaagcgtcttgctcctctgtcaagctcctccttgccactcttggccgcctgcaaagccgcctccaagatgatcttctcgttctgcaggaggcagatcgtgtcctccctggaggcggcctcgccctgcagctcccccagcctggcctgcagctcatcgtagtgtgtctgcagggcatcgagggactgctccctgctctgcagagcctcctgagtcaaggtgagctgtttcatcaggtccaggtgctcctgctgcaaagcctcaagctgctggtctcgctggagtaaagtcaacttcacctgctccagctgctgctccagggatgccgccgagtccgccatcctctgcagccgctccctctcaccttcaaactcttccagcctcctctgaaggtcctcctccaccatcgtctttgcctcctgaatctgcatgaaggctgcttcctgatccaacatgtcagcctcaatgccctgcagctgtgccgcgatgcgccccttctccttcatggacctgtgctgagtttccgtcagctgctgggacagggacacattctcgagtttcaggtgctccaggagacctgcctgggtcatctgtccaacctggatgtgggccatctcaccctgcagcctgacgcgggcctcctgtgccagggcgagctgctgctggtaccactgccggacactctgcagggacgagatctccgcctgcgacgccttcagcttgctggtcagcgtcgtccgctccagctgcacctgctgaagctggctctgcaaggctgtcatctgctgtcgcaggtcgtgcactgtgttgtccttgctgagcatgctcctctgcatgtcctctaccttggccataagcctctggtactgctcctcggccacctgcaagtcgttgttggacgacgccaggctggcattttttgcctccagcatgttctgcaggtcagtcatggctcgctccaggtcccagcacgactgcttcagggtgtccacctccgagctcagcgaatcctgccgctgctggctgctgtggctgcactccacctgcgcctgcagcttcgtgctgagggcggccagctgggcctgcagctcagccttctctttaagtgcctgactcgcctccagtgacaaggcttccagctgtccttcgagtcgcattttctctttgagcacctgcagcatctcctcctgtgtttctgctgcagagctctccaaggacacgctgctgcagatgctgtctctccgactccgcacctccccgttgacctcctgcccctggtcttggtgctcagcggctgcggcctggaggacgtccttaatggaggggaactggcccagggtatccgcaggaatctcctggccgttgaccatatagggggtgtcctgcgtgcccactgtcttcgacagaatgccataggtccctcgggtggaggcgctgctgtacgatgagctgtcgctgtcatttccatccacctcagacacgctgtctccagccagggaggtgttctccagacggtcgtcagtgtcgggggacaggctgatctcagacacaacggacgccgcactgcttctgttctgcttcagggaacccttggtagaatcgggagccgggacatttcccccagaattccccgcatttgaatcttcagttctgtaatcggccagagaccggattttgcttgatttggaagtttttttctccctaggatgtgccggaagccccaggctgcccaccttaggcccccgagggacactggtgcgcaggaaggaatattcttttgtcatagccagggtactggcccttggtaagttttctgggtttaacatgagctcaggatcaagcgtgctaaaaagtctcgttttggttgcaggttgactggacctctcctgctggcgcttcaccctgtactgtttgagctgctcttccagccacttccgagcctgaagtcggacctgctcctccttctccaggggcaggggagaatctgtagagcacagttgcgtttcttgcataggaagactgagtctgagagactgcaaagcttcttttctaacactgccctcagcactagttccctgagacttccttaggttgtcatggaaaccagccacacctggagaggcatcagggcccactgggcttgtggtgggatcgagagacgacggagggtctgggaagggtggcgttggcccgttctgacagaggcctccctggccaggtccatccgggctttccccttccgtggatgctctgtttacctcggcacactggactttgtcctgctggtcaggtggcaccagtgggcccgggggcttcagtggggcctcggggagagacgaggggccactgtgggatctgtcctcctggaggccatcttgctcggccgacgcgccgtccatggtcaggacgacaccagctgagctgacgctgaggggctacaagtgaaccttggacaagcttggcttctgccatcagcaacagccaagagctcctgggaggggccctactgtgtctcccattttcaggagaagatctgatgactcacaaatgacttgatgtcaaaccagctaatatcatgatacttgggaaagtatgctacttcttaaggcaatcgggggaaaaaaagctcctcttcaatctgagtgatgtcagatgatttatttccttcttgccatttaaggtatactgccctgctgctctggcagcc

SEQ ID NO: 14313 - RNA, 7035 nt, Homo sapiens
  source 1..7035: mol_type = other RNA
gctgggattacaggcatgagccaccgcgcccggcccgatttcttgattttaaaattaaaacaaaggggtagtacagccaaaataaataagaacgtaaattgccgtatttttttttctaatggtacaagaacaatttagtaaataacatcttcaacttaagataaaaagtaggatatatttataatgaaattttcaagtattatttcaaaattaaccctgtacaaatgatatattttggaaattccaatatttgctagagaatattttttaaataccaaacatctttgtggttaatgctaccttaaccttaccaattaaccttctaaaagtatattacaacagaacacaaatagcttaaaacacaccatactgttttctccacaaaacagacaccagacaccgacatgagcacatctggcctggccagtgactcagaacctcatttcagaccagtacatctgcagaggaggccacgcggacccattctctctctcctaactcatataataaatattattttagattttcttagcaaactaggggacaacttacagaccccacctctcccagtcagccagtgtctgcagggtttcaggatttggggtaggaaacagaagatctcacacatgtcgtgctgattttaaataaggcatctgtctctgagacacctgggagagcacagccaccttcctcacggtgcctgcctgtctcttccggaagtcgcctctgcttgccacatgatgctggtgtaaccacaaaagatccaggacttctcgatgactgcagaagtacaggtgctcctacacacgagtacaggcgctcccacagacaatggtaaagattttcacttggggaacaggagtgtgaggtttgttaccgcctgcgacctacacctggctgactccaggggaaaccgcgggagtcgctgcagggagcccctggtctgctctcctcctcctcctccaccggcctctccctgtgcccccccaaaggtcagatcagatatggggcctcagtgtccttgtgcctcctgatggccgtcaggcctgaccaagggtccaagctgccccttcccagtggccagccacggtggaatcacacagggccagtggcctgagaggaagagaccagcaggaaggaaagatcctcagcaacaaagtaaaaccagaacaacagaggacctttctgtgtaagaatatttggctttagaaggtaaataaaataattatatttcttagaattttctgactatccctaaatcctgcaggtaaattattcccaacaaattttcaaaaggcaatcaataataagtaggttcttcttcaataacatgagcatatgcttcttaaagactgggtgacaggccgggcgcaggggctcacgcctgtaatcccagcactttgggaggctgagatgggcagatcacttgaggtcaggagatcgagaccatcctggccaacatggtgaaaccccattgctactaaaaatacaaacattagcctggcatagtggcgcacgcctgtaatcccagctactcgagaggctgaggcaggagaatcgcatgaacctgggaggcggagcttgcagtgagcggagagtgtgccactgcactccagcctgggcaacaaagcgagactctgtctcaaaaaaaaaaaaaaaaaaaaaacaaagattggattatgatattcagtatctatgtacacatcctatggtgggatggctatccaaaaaaacaagtaaaaagccaaaggtacagataaaatttcatttctgcggaaaagtaaagctcttactgaatggaacagggaagtgagaaactgcagccggcctggccaggcgcggtgccgcagaccctgtcacacagctgctcccagttacgcagcctctccctgtcacccgcagagagcagcatcggtggccgctcagaagccacgacctacaagtaacccttcagacacgttcaaagctcctcgccgagagcctatcaggcttttaagagttggtcattccatgtgaaaagctaattgtgatcttcgaatgtttttctagtccttggctctcattctgctatatattttacttcttgttaaaggcaaaacaaaacttaaatttcatgtcttagaaaaacatcgaccacacaatcaaataaataacattgataagagccttctggggcagcggcgcacggaggcgagtccacagcagtcactctcccggcccttctttggaagccctgctctgactgtgtctctgtgggtcgccgcgtgggccggcgtgaccccccgggggcacagggctggcagtggctggctccagcggcgtccacgaggacagagactcgtgcaccgtcagggcgtgctcctccatctggcgctgcaggctgtccatctcctgcttgagctgctggaggcagctgttcaggttcttgaggggctccttgctcacggcgggcggtggtctcagcagctcctccagcagcgaggcgggaactgggcagtccgggatcttgatgggcgtggcagggttggaagagctggcctcgcctttcggctcctttctcgtcttggccgcgccgcggcgtaggtccagcttgagctgctggttctgctggagcagggtcttcatgttgttcttcagctccgacacttttgcctggagcataaatttatccttctgggtcatggacaggtcttcctgggccatctccaactcagacttgacgttctgcagcagctgctgtagcccttccagttccttcctgccctgctgctccgtcaagtccagctgctgcttcaaggactggatttctctttctttctgatccacctcccatttgagattttccatctcttggtttcccacgggctgtttgctgagctgctcgtccagctgcttctgcaggagctggagctgtgcccgggcctcggccagctctgcttggaactgtgctatctcctgggaatgtttcccctcccgaatctgaaggtcgtcggcctcggcctgcagcttctgcaccaggtgttccttggcctgcagctccttcttcacctcactcagctccaaggaggccgccttgaagtggcggcggttatgcccggcttccaccttggcagcagccacctgctccttgaggctgttcaccttctccttctccttctctagtgaggcctgcagggcctggacaagatgcttcatctggcgatcctcctcttctttgcgctgcaaaactgcctgcacctgaaggttcaactggactaggtctgcctccctcttggccaaagctgtttctaggatgctgttgtgttcccgcagagctgcgttggactgaccgaggcccgtaagcttccctttctcgtgctctaattcaagagccaacttcttgtttgactcctcaaggcgttttatcttcttcctaaagcctctggattcttgaagctcgtcctccagctccagcaccttctcccgggactcctccagctcctggctggtcagcgctatgacctcctgcagttccttttccagcagcgtcttgctatgactgacagcctgcagctccgcctccagggcctggatcctttcatgtagagccaggctgctgtcactgctgccaccctgggctcggagctggcccagctccgcgtccgcagcctccttggccgcgagggcctcctgcaggcggcggctgaggatgcccacggcgttctcgtaggccttatgtttggtcttcatctccttctgggcgctggtcaagtctgagcccagccgcctcatcttctgcttctgttccgtgatggccttccgggcctcttgctgcaactcttcgatttgtttcttcagcgcctcattggcctctgtgaccgcgaccatctgctccttatcgaactgcaacgactgcaagtgtgtttccatctcgtctcgctccttctgcgccgactggagatgcccttcaaggtccgccatgtgctgacggacctgggccacctctctgtgcaggcgcgagagctccgcctcggcagtccgcttctccccgtgcacttgcatcagctcctgccgcagctccttcagctccgagtccagcctcttcctggtggctttcagctcactgatgagctggtctttggaggtggcgtcgcgccggtaggcctccaccatcaccttttgttggagaaactgttcctttattttttgcatttgctttttcagagcagcagtctcctgctgcaggtgttccacctggccggatttgatagctaattcttctcttaacttctctaaagtttccgacgtttcctcggtaccttcttccaagcgtcttgctcctctgtcaagctcctccttgccactcttggccgcctgcaaagccgcctccaagatgatcttctcgttctgcaggaggcagatcgtgtcctccctggaggcggcctcgccctgcagctcccccagcctggcctgcagctcatcgtagtgtgtctgcagggcatcgagggactgctccctgctctgcagagcctcctgagtcaaggtgagctgtttcatcaggtccaggtgctcctgctgcaaagcctcaagctgctggtctcgctggagtaaagtcaacttcacctgctccagctgctgctccagggatgccgccgagtccgccatcctctgcagccgctccctctcaccttcaaactcttccagcctcctctgaaggtcctcctccaccatcgtctttgcctcctgaatctgcatgaaggctgcttcctgatccaacatgtcagcctcaatgccctgcagctgtgccgcgatgcgccccttctccttcatggacctgtgctgagtttccgtcagctgctgggacagggacacattctcgagtttcaggtgctccaggagacctgcctgggtcatctgtccaacctggatgtgggccatctcaccctgcagcctgacgcgggcctcctgtgccagggcgagctgctgctggtaccactgccggacactctgcagggacgagatctccgcctgcgacgccttcagcttgctggtcagcgtcgtccgctccagctgcacctgctgaagctggctctgcaaggctgtcatctgctgtcgcaggtcgtgcactgtgttgtccttgctgagcatgctcctctgcatgtcctctaccttggccataagcctctggtactgctcctcggccacctgcaagtcgttgttggacgacgccaggctggcattttttgcctccagcatgttctgcaggtcagtcatggctcgctccaggtcccagcacgactgcttcagggtgtccacctccgagctcagcgaatcctgccgctgctggctgctgtggctgcactccacctgcgcctgcagcttcgtgctgagggcggccagctgggcctgcagctcagccttctctttaagtgcctgactcgcctccagtgacaaggcttccagctgtccttcgagtcgcattttctctttgagcacctgcagcatctcctcctgtgtttctgctgcagagctctccaaggacacgctgctgcagatgctgtctctccgactccgcacctccccgttgacctcctgcccctggtcttggtgctcagcggctgcggcctggaggacgtccttaatggaggggaactggcccagggtatccgcaggaatctcctggccgttgaccatatagggggtgtcctgcgtgcccactgtcttcgacagaatgccataggtccctcgggtggaggcgctgctgtacgatgagctgtcgctgtcatttccatccacctcagacacgctgtctccagccagggaggtgttctccagacggtcgtcagtgtcgggggacaggctgatctcagacacaacggacgccgcactgcttctgttctgcttcagggaacccttggtagaatcgggagccgggacatttcccccagaattccccgcatttgaatcttcagttctgtaatcggccagagaccggattttgcttgatttggaagtttttttctccctaggatgtgccggaagccccaggctgcccaccttaggcccccgagggacactggtgcgcaggaaggaatattcttttgtcatagccagggtactggcccttggtaagttttctgggtttaacatgagctcaggatcaagcgtgctaaaaagtctcgttttggttgcaggttgactggacctctcctgctggcgcttcaccctgtactgtttgagctgctcttccagccacttccgagcctgaagtcggacctgctcctccttctccaggggcaggggagaatctgtagagcacagttgcgtttcttgcataggaagactgagtctgagagactgcaaagcttcttttctaacactgccctcagcactagttccctgagacttccttaggttgtcatggaaaccagccacacctggagaggcatcagggcccactgggcttgtggtgggatcgagagacgacggagggtctgggaagggtggcgttggcccgttctgacagaggcctccctggccaggtccatccgggctttccccttccgtggatgctctgtttacctcggcacactggactttgtcctgctggtcaggtggcaccagtgggcccgggggcttcagtggggcctcggggagagacgaggggccactgtgggatctgtcctcctggaggccatcttgctcggccgacgcgccgtccatggtcaggacgacaccagctgagctgacgctgaggggctacaagtgaaccttggacaagcttggcttctgccatcagcaacagccaagagctcctgggaggggccctactgtgtctcccattttcaggagaagatctgatgactcacaaatgacttgatgtcaaaccagctaatatcatgatacttgggaaagtatgctacttcttaaggcaatcgggggaaaaaaagctcctcttcaatctgagtgatgtcagatgatttatttccttcttgccatttaaggtatactgcctgtaacaccagcactttgggaggctggggtgggaggatcgct

SEQ ID NO: 14314 - RNA, 6715 nt, Homo sapiens
  source 1..6715: mol_type = other RNA
gctgggattacaggcatgagccaccgcgcccggcccgatttcttgattttaaaattaaaacaaaggggtagtacagccaaaataaataagaacgtaaattgccgtatttttttttctaatggtacaagaacaatttagtaaataacatcttcaacttaagataaaaagtaggatatatttataatgaaattttcaagtattatttcaaaattaaccctgtacaaatgatatattttggaaattccaatatttgctagagaatattttttaaataccaaacatctttgtggttaatgctaccttaaccttaccaattaaccttctaaaagtatattacaacagaacacaaatagcttaaaacacaccatactgttttctccacaaaacagacaccagacaccgacatgagcacatctggcctggccagtgactcagaacctcatttcagaccagtacatctgcagaggaggccacgcggacccattctctctctcctaactcatataataaatattattttagattttcttagcaaactaggggacaacttacagaccccacctctcccagtcagccagtgtctgcagggtttcaggatttggggtaggaaacagaagatctcacacatgtcgtgctgattttaaataaggcatctgtctctgagacacctgggagagcacagccaccttcctcacggtgcctgcctgtctcttccggaagtcgcctctgcttgccacatgatgctggtgtaaccacaaaagatccaggacttctcgatgactgcagaagtacaggtgctcctacacacgagtacaggcgctcccacagacaatggtaaagattttcacttggggaacaggagtgtgaggtttgttaccgcctgcgacctacacctggctgactccaggggaaaccgcgggagtcgctgcagggagcccctggtctgctctcctcctcctcctccaccggcctctccctgtgcccccccaaaggtcagatcagatatggggcctcagtgtccttgtgcctcctgatggccgtcaggcctgaccaagggtccaagctgccccttcccagtggccagccacggtggaatcacacagggccagtggcctgagaggaagagaccagcaggaaggaaagatcctcagcaacaaagtaaaaccagaacaacagaggacctttctgtgtaagaatatttggctttagaaggtaaataaaataattatatttcttagaattttctgactatccctaaatcctgcaggtaaattattcccaacaaattttcaaaaggcaatcaataataagtaggttcttcttcaataacatgagcatatgcttcttaaagactgggtgacaggccgggcgcaggggctcacgcctgtaatcccagcactttgggaggctgagatgggcagatcacttgaggtcaggagatcgagaccatcctggccaacatggtgaaaccccattgctactaaaaatacaaacattagcctggcatagtggcgcacgcctgtaatcccagctactcgagaggctgaggcaggagaatcgcatgaacctgggaggcggagcttgcagtgagcggagagtgtgccactgcactccagcctgggcaacaaagcgagactctgtctcaaaaaaaaaaaaaaaaaaaaaacaaagattggattatgatattcagtatctatgtacacatcctatggtgggatggctatccaaaaaaacaagtaaaaagccaaaggtacagataaaatttcatttctgcggaaaagtaaagctcttactgaatggaacagggaagtgagaaactgcagccggcctggccaggcgcggtgccgcagaccctgtcacacagctgctcccagttacgcagcctctccctgtcacccgcagagagcagcatcggtggccgctcagaagccacgacctacaagtaacccttcagacacgttcaaagctcctcgccgagagcctatcaggcttttaagagttggtcattccatgtgaaaagctaattgtgatcttcgaatgtttttctagtccttggctctcattctgctatatattttacttcttgttaaaggcaaaacaaaacttaaatttcatgtcttagaaaaacatcgaccacacaatcaaataaataacattgataagagccttctggggcagcggcgcacggaggcgagtccacagcagtcactctcccggcccttctttggaagccctgctctgactgtgtctctgtgggtcgccgcgtgggccggcgtgaccccccgggggcacagggctggcagtggctggctccagcggcgtccacgaggacagagactcgtgcaccgtcagggcgtgctcctccatctggcgctgcaggctgtccatctcctgcttgagctgctggaggcagctgttcaggttcttgaggggctccttgctcacggcgggcggtggtctcagcagctcctccagcagcgaggcgggaactgggcagtccgggatcttgatgggcgtggcagggttggaagagctggcctcgcctttcggctcctttctcgtcttggccgcgccgcggcgtaggtccagcttgagctgctggttctgctggagcagggtcttcatgttgttcttcagctccgacacttttgcctggagcataaatttatccttctgggtcatggacaggtcttcctgggccatctccaactcagacttgacgttctgcagcagctgctgtagcccttccagttccttcctgccctgctgctccgtcaagtccagctgctgcttcaaggactggatttctctttctttctgatccacctcccatttgagattttccatctcttggtttcccacgggctgtttgctgagctgctcgtccagctgcttctgcaggagctggagctgtgcccgggcctcggccagctctgcttggaactgtgctatctcctgggaatgtttcccctcccgaatctgaaggtcgtcggcctcggcctgcagcttctgcaccaggtgttccttggcctgcagctccttcttcacctcactcagctccaaggaggccgccttgaagtggcggcggttatgcccggcttccaccttggcagcagccacctgctccttgaggctgttcaccttctccttctccttctctagtgaggcctgcagggcctggacaagatgcttcatctggcgatcctcctcttctttgcgctgcaaaactgcctgcacctgaaggttcaactggactaggtctgcctccctcttggccaaagctgtttctaggatgctgttgtgttcccgcagagctgcgttggactgaccgaggcccgtaagcttccctttctcgtgctctaattcaagagccaacttcttgtttgactcctcaaggcgttttatcttcttcctaaagcctctggattcttgaagctcgtcctccagctccagcaccttctcccgggactcctccagctcctggctggtcagcgctatgacctcctgcagttccttttccagcagcgtcttgctatgactgacagcctgcagctccgcctccagggcctggatcctttcatgtagagccaggctgctgtcactgctgccaccctgggctcggagctggcccagctccgcgtccgcagcctccttggccgcgagggcctcctgcaggcggcggctgaggatgcccacggcgttctcgtaggccttatgtttggtcttcatctccttctgggcgctggtcaagtctgagcccagccgcctcatcttctgcttctgttccgtgatggccttccgggcctcttgctgcaactcttcgatttgtttcttcagcgcctcattggcctctgtgaccgcgaccatctgctccttatcgaactgcaacgactgcaagtgtgtttccatctcgtctcgctccttctgcgccgactggagatgcccttcaaggtccgccatgtgctgacggacctgggccacctctctgtgcaggcgcgagagctccgcctcggcagtccgcttctccccgtgcacttgcatcagctcctgccgcagctccttcagctccgagtccagcctcttcctggtggctttcagctcactgatgagctggtctttggaggtggcgtcgcgccggtaggcctccaccatcaccttttgttggagaaactgttcctttattttttgcatttgctttttcagagcagcagtctcctgctgcaggtgttccacctggccggatttgatagctaattcttctcttaacttctctaaagtttccgacgtttcctcggtaccttcttccaagcgtcttgctcctctgtcaagctcctccttgccactcttggccgcctgcaaagccgcctccaagatgatcttctcgttctgcaggaggcagatcgtgtcctccctggaggcggcctcgccctgcagctcccccagcctggcctgcagctcatcgtagtgtgtctgcagggcatcgagggactgctccctgctctgcagagcctcctgagtcaaggtgagctgtttcatcaggtccaggtgctcctgctgcaaagcctcaagctgctggtctcgctggagtaaagtcaacttcacctgctccagctgctgctccagggatgccgccgagtccgccatcctctgcagccgctccctctcaccttcaaactcttccagcctcctctgaaggtcctcctccaccatcgtctttgcctcctgaatctgcatgaaggctgcttcctgatccaacatgtcagcctcaatgccctgcagctgtgccgcgatgcgccccttctccttcatggacctgtgctgagtttccgtcagctgctgggacagggacacattctcgagtttcaggtgctccaggagacctgcctgggtcatctgtccaacctggatgtgggccatctcaccctgcagcctgacgcgggcctcctgtgccagggcgagctgctgctggtaccactgccggacactctgcagggacgagatctccgcctgcgacgccttcagcttgctggtcagcgtcgtccgctccagctgcacctgctgaagctggctctgcaaggctgtcatctgctgtcgcaggtcgtgcactgtgttgtccttgctgagcatgctcctctgcatgtcctctaccttggccataagcctctggtactgctcctcggccacctgcaagtcgttgttggacgacgccaggctggcattttttgcctccagcatgttctgcaggtcagtcatggctcgctccaggtcccagcacgactgcttcagggtgtccacctccgagctcagcgaatcctgccgctgctggctgctgtggctgcactccacctgcgcctgcagcttcgtgctgagggcggccagctgggcctgcagctcagccttctctttaagtgcctgactcgcctccagtgacaaggcttccagctgtccttcgagtcgcattttctctttgagcacctgcagcatctcctcctgtgtttctgctgcagagctctccaaggacacgctgctgcagatgctgtctctccgactccgcacctccccgttgacctcctgcccctggtcttggtgctcagcggctgcggcctggaggacgtccttaatggaggggaactggcccagggtatccgcaggaatctcctggccgttgaccatatagggggtgtcctgcgtgcccactgtcttcgacagaatgccataggtccctcgggtggaggcgctgctgtacgatgagctgtcgctgtcatttccatccacctcagacacgctgtctccagccagggaggtgttctccagacggtcgtcagtgtcgggggacaggctgatctcagacacaacggacgccgcactgcttctgttctgcttcagggaacccttggtagaatcgggagccgggacatttcccccagaattccccgcatttgaatcttcagttctgtaatcggccagagaccggattttgcttgatttggaagtttttttctccctaggatgtgccggaagccccaggctgcccaccttaggcccccgagggacactggtgcgcaggaaggaatattcttttgtcatagccagggtactggcccttggtaagttttctgggtttaacatgagctcaggatcaagcgtgctaaaaagtctcgttttggttgcaggttgactggacctctcctgctggcgcttcaccctgtactgtttgagctgctcttccagccacttccgagcctgaagtcggacctgctcctccttctccaggggcaggggagaatctgtagagcactggactttgtcctgctggtcaggtggcaccagtgggcccgggggcttcagtggggcctcggggagagacgaggggccactgtgggatctgtcctcctggaggccatcttgctcggccgacgcgccgtccatggtcaggacgacaccagctgagctgacgctgaggggctacaagtgaaccttggacaagcttggcttctgccatcagcaacagccaagagctcctgggaggggccctactgtgtctcccattttcaggagaagatctgatgactcacaaatgacttgatgtcaaaccagctaatatcatgataccctgctgctctggcagccccggaggccgcccggcccggatgctccggcggagacgtggccgtgagaggggcggggcgagcggtgcatcggcctcgggtccccg

SEQ ID NO: 14315 - RNA, 6868 nt, Homo sapiens
  source 1..6868: mol_type = other RNA
gctgggattacaggcatgagccaccgcgcccggcccgatttcttgattttaaaattaaaacaaaggggtagtacagccaaaataaataagaacgtaaattgccgtatttttttttctaatggtacaagaacaatttagtaaataacatcttcaacttaagataaaaagtaggatatatttataatgaaattttcaagtattatttcaaaattaaccctgtacaaatgatatattttggaaattccaatatttgctagagaatattttttaaataccaaacatctttgtggttaatgctaccttaaccttaccaattaaccttctaaaagtatattacaacagaacacaaatagcttaaaacacaccatactgttttctccacaaaacagacaccagacaccgacatgagcacatctggcctggccagtgactcagaacctcatttcagaccagtacatctgcagaggaggccacgcggacccattctctctctcctaactcatataataaatattattttagattttcttagcaaactaggggacaacttacagaccccacctctcccagtcagccagtgtctgcagggtttcaggatttggggtaggaaacagaagatctcacacatgtcgtgctgattttaaataaggcatctgtctctgagacacctgggagagcacagccaccttcctcacggtgcctgcctgtctcttccggaagtcgcctctgcttgccacatgatgctggtgtaaccacaaaagatccaggacttctcgatgactgcagaagtacaggtgctcctacacacgagtacaggcgctcccacagacaatggtaaagattttcacttggggaacaggagtgtgaggtttgttaccgcctgcgacctacacctggctgactccaggggaaaccgcgggagtcgctgcagggagcccctggtctgctctcctcctcctcctccaccggcctctccctgtgcccccccaaaggtcagatcagatatggggcctcagtgtccttgtgcctcctgatggccgtcaggcctgaccaagggtccaagctgccccttcccagtggccagccacggtggaatcacacagggccagtggcctgagaggaagagaccagcaggaaggaaagatcctcagcaacaaagtaaaaccagaacaacagaggacctttctgtgtaagaatatttggctttagaaggtaaataaaataattatatttcttagaattttctgactatccctaaatcctgcaggtaaattattcccaacaaattttcaaaaggcaatcaataataagtaggttcttcttcaataacatgagcatatgcttcttaaagactgggtgacaggccgggcgcaggggctcacgcctgtaatcccagcactttgggaggctgagatgggcagatcacttgaggtcaggagatcgagaccatcctggccaacatggtgaaaccccattgctactaaaaatacaaacattagcctggcatagtggcgcacgcctgtaatcccagctactcgagaggctgaggcaggagaatcgcatgaacctgggaggcggagcttgcagtgagcggagagtgtgccactgcactccagcctgggcaacaaagcgagactctgtctcaaaaaaaaaaaaaaaaaaaaaacaaagattggattatgatattcagtatctatgtacacatcctatggtgggatggctatccaaaaaaacaagtaaaaagccaaaggtacagataaaatttcatttctgcggaaaagtaaagctcttactgaatggaacagggaagtgagaaactgcagccggcctggccaggcgcggtgccgcagaccctgtcacacagctgctcccagttacgcagcctctccctgtcacccgcagagagcagcatcggtggccgctcagaagccacgacctacaagtaacccttcagacacgttcaaagctcctcgccgagagcctatcaggcttttaagagttggtcattccatgtgaaaagctaattgtgatcttcgaatgtttttctagtccttggctctcattctgctatatattttacttcttgttaaaggcaaaacaaaacttaaatttcatgtcttagaaaaacatcgaccacacaatcaaataaataacattgataagagccttctggggcagcggcgcacggaggcgagtccacagcagtcactctcccggcccttctttggaagccctgctctgactgtgtctctgtgggtcgccgcgtgggccggcgtgaccccccgggggcacagggctggcagtggctggctccagcggcgtccacgaggacagagactcgtgcaccgtcagggcgtgctcctccatctggcgctgcaggctgtccatctcctgcttgagctgctggaggcagctgttcaggttcttgaggggctccttgctcacggcgggcggtggtctcagcagctcctccagcagcgaggcgggaactgggcagtccgggatcttgatgggcgtggcagggttggaagagctggcctcgcctttcggctcctttctcgtcttggccgcgccgcggcgtaggtccagcttgagctgctggttctgctggagcagggtcttcatgttgttcttcagctccgacacttttgcctggagcataaatttatccttctgggtcatggacaggtcttcctgggccatctccaactcagacttgacgttctgcagcagctgctgtagcccttccagttccttcctgccctgctgctccgtcaagtccagctgctgcttcaaggactggatttctctttctttctgatccacctcccatttgagattttccatctcttggtttcccacgggctgtttgctgagctgctcgtccagctgcttctgcaggagctggagctgtgcccgggcctcggccagctctgcttggaactgtgctatctcctgggaatgtttcccctcccgaatctgaaggtcgtcggcctcggcctgcagcttctgcaccaggtgttccttggcctgcagctccttcttcacctcactcagctccaaggaggccgccttgaagtggcggcggttatgcccggcttccaccttggcagcagccacctgctccttgaggctgttcaccttctccttctccttctctagtgaggcctgcagggcctggacaagatgcttcatctggcgatcctcctcttctttgcgctgcaaaactgcctgcacctgaaggttcaactggactaggtctgcctccctcttggccaaagctgtttctaggatgctgttgtgttcccgcagagctgcgttggactgaccgaggcccgtaagcttccctttctcgtgctctaattcaagagccaacttcttgtttgactcctcaaggcgttttatcttcttcctaaagcctctggattcttgaagctcgtcctccagctccagcaccttctcccgggactcctccagctcctggctggtcagcgctatgacctcctgcagttccttttccagcagcgtcttgctatgactgacagcctgcagctccgcctccagggcctggatcctttcatgtagagccaggctgctgtcactgctgccaccctgggctcggagctggcccagctccgcgtccgcagcctccttggccgcgagggcctcctgcaggcggcggctgaggatgcccacggcgttctcgtaggccttatgtttggtcttcatctccttctgggcgctggtcaagtctgagcccagccgcctcatcttctgcttctgttccgtgatggccttccgggcctcttgctgcaactcttcgatttgtttcttcagcgcctcattggcctctgtgaccgcgaccatctgctccttatcgaactgcaacgactgcaagtgtgtttccatctcgtctcgctccttctgcgccgactggagatgcccttcaaggtccgccatgtgctgacggacctgggccacctctctgtgcaggcgcgagagctccgcctcggcagtccgcttctccccgtgcacttgcatcagctcctgccgcagctccttcagctccgagtccagcctcttcctggtggctttcagctcactgatgagctggtctttggaggtggcgtcgcgccggtaggcctccaccatcaccttttgttggagaaactgttcctttattttttgcatttgctttttcagagcagcagtctcctgctgcaggtgttccacctggccggatttgatagctaattcttctcttaacttctctaaagtttccgacgtttcctcggtaccttcttccaagcgtcttgctcctctgtcaagctcctccttgccactcttggccgcctgcaaagccgcctccaagatgatcttctcgttctgcaggaggcagatcgtgtcctccctggaggcggcctcgccctgcagctcccccagcctggcctgcagctcatcgtagtgtgtctgcagggcatcgagggactgctccctgctctgcagagcctcctgagtcaaggtgagctgtttcatcaggtccaggtgctcctgctgcaaagcctcaagctgctggtctcgctggagtaaagtcaacttcacctgctccagctgctgctccagggatgccgccgagtccgccatcctctgcagccgctccctctcaccttcaaactcttccagcctcctctgaaggtcctcctccaccatcgtctttgcctcctgaatctgcatgaaggctgcttcctgatccaacatgtcagcctcaatgccctgcagctgtgccgcgatgcgccccttctccttcatggacctgtgctgagtttccgtcagctgctgggacagggacacattctcgagtttcaggtgctccaggagacctgcctgggtcatctgtccaacctggatgtgggccatctcaccctgcagcctgacgcgggcctcctgtgccagggcgagctgctgctggtaccactgccggacactctgcagggacgagatctccgcctgcgacgccttcagcttgctggtcagcgtcgtccgctccagctgcacctgctgaagctggctctgcaaggctgtcatctgctgtcgcaggtcgtgcactgtgttgtccttgctgagcatgctcctctgcatgtcctctaccttggccataagcctctggtactgctcctcggccacctgcaagtcgttgttggacgacgccaggctggcattttttgcctccagcatgttctgcaggtcagtcatggctcgctccaggtcccagcacgactgcttcagggtgtccacctccgagctcagcgaatcctgccgctgctggctgctgtggctgcactccacctgcgcctgcagcttcgtgctgagggcggccagctgggcctgcagctcagccttctctttaagtgcctgactcgcctccagtgacaaggcttccagctgtccttcgagtcgcattttctctttgagcacctgcagcatctcctcctgtgtttctgctgcagagctctccaaggacacgctgctgcagatgctgtctctccgactccgcacctccccgttgacctcctgcccctggtcttggtgctcagcggctgcggcctggaggacgtccttaatggaggggaactggcccagggtatccgcaggaatctcctggccgttgaccatatagggggtgtcctgcgtgcccactgtcttcgacagaatgccataggtccctcgggtggaggcgctgctgtacgatgagctgtcgctgtcatttccatccacctcagacacgctgtctccagccagggaggtgttctccagacggtcgtcagtgtcgggggacaggctgatctcagacacaacggacgccgcactgcttctgttctgcttcagggaacccttggtagaatcgggagccgggacatttcccccagaattccccgcatttgaatcttcagttctgtaatcggccagagaccggattttgcttgatttggaagtttttttctccctaggatgtgccggaagccccaggctgcccaccttaggcccccgagggacactggtgcgcaggaaggaatattcttttgtcatagccagggtactggcccttggtaagttttctgggtttaacatgagctcaggatcaagcgtgctaaaaagtctcgttttggttgcaggttgactggacctctcctgctggcgcttcaccctgtactgtttgagctgctcttccagccacttccgagcctgaagtcggacctgctcctccttctccaggggcaggggagaatctgtagagcctggagaggcatcagggcccactgggcttgtggtgggatcgagagacgacggagggtctgggaagggtggcgttggcccgttctgacagaggcctccctggccaggtccatccgggctttccccttccgtggatgctctgtttacctcggcacactggactttgtcctgctggtcaggtggcaccagtgggcccgggggcttcagtggggcctcggggagagacgaggggccactgtgggatctgtcctcctggaggccatcttgctcggccgacgcgccgtccatggtcaggacgacaccagctgagctgacgctgaggggctacaagtgaaccttggacaagcttggcttctgccatcagcaacagccaagagctcctgggaggggccctactgtgtctcccattttcaggagaagatctgatgactcacaaatgacttgatgtcaaaccagctaatatcatgataccctgctgctctggcagccccggaggccgcccggcccggatgctccggcggagacgtggccgtgagaggggcggggcgagcggtgcatcggcctcgggtccccg

SEQ ID NO: 14316 - RNA, 6878 nt, Homo sapiens
  source 1..6878: mol_type = other RNA
gctgggattacaggcatgagccaccgcgcccggcccgatttcttgattttaaaattaaaacaaaggggtagtacagccaaaataaataagaacgtaaattgccgtatttttttttctaatggtacaagaacaatttagtaaataacatcttcaacttaagataaaaagtaggatatatttataatgaaattttcaagtattatttcaaaattaaccctgtacaaatgatatattttggaaattccaatatttgctagagaatattttttaaataccaaacatctttgtggttaatgctaccttaaccttaccaattaaccttctaaaagtatattacaacagaacacaaatagcttaaaacacaccatactgttttctccacaaaacagacaccagacaccgacatgagcacatctggcctggccagtgactcagaacctcatttcagaccagtacatctgcagaggaggccacgcggacccattctctctctcctaactcatataataaatattattttagattttcttagcaaactaggggacaacttacagaccccacctctcccagtcagccagtgtctgcagggtttcaggatttggggtaggaaacagaagatctcacacatgtcgtgctgattttaaataaggcatctgtctctgagacacctgggagagcacagccaccttcctcacggtgcctgcctgtctcttccggaagtcgcctctgcttgccacatgatgctggtgtaaccacaaaagatccaggacttctcgatgactgcagaagtacaggtgctcctacacacgagtacaggcgctcccacagacaatggtaaagattttcacttggggaacaggagtgtgaggtttgttaccgcctgcgacctacacctggctgactccaggggaaaccgcgggagtcgctgcagggagcccctggtctgctctcctcctcctcctccaccggcctctccctgtgcccccccaaaggtcagatcagatatggggcctcagtgtccttgtgcctcctgatggccgtcaggcctgaccaagggtccaagctgccccttcccagtggccagccacggtggaatcacacagggccagtggcctgagaggaagagaccagcaggaaggaaagatcctcagcaacaaagtaaaaccagaacaacagaggacctttctgtgtaagaatatttggctttagaaggtaaataaaataattatatttcttagaattttctgactatccctaaatcctgcaggtaaattattcccaacaaattttcaaaaggcaatcaataataagtaggttcttcttcaataacatgagcatatgcttcttaaagactgggtgacaggccgggcgcaggggctcacgcctgtaatcccagcactttgggaggctgagatgggcagatcacttgaggtcaggagatcgagaccatcctggccaacatggtgaaaccccattgctactaaaaatacaaacattagcctggcatagtggcgcacgcctgtaatcccagctactcgagaggctgaggcaggagaatcgcatgaacctgggaggcggagcttgcagtgagcggagagtgtgccactgcactccagcctgggcaacaaagcgagactctgtctcaaaaaaaaaaaaaaaaaaaaaacaaagattggattatgatattcagtatctatgtacacatcctatggtgggatggctatccaaaaaaacaagtaaaaagccaaaggtacagataaaatttcatttctgcggaaaagtaaagctcttactgaatggaacagggaagtgagaaactgcagccggcctggccaggcgcggtgccgcagaccctgtcacacagctgctcccagttacgcagcctctccctgtcacccgcagagagcagcatcggtggccgctcagaagccacgacctacaagtaacccttcagacacgttcaaagctcctcgccgagagcctatcaggcttttaagagttggtcattccatgtgaaaagctaattgtgatcttcgaatgtttttctagtccttggctctcattctgctatatattttacttcttgttaaaggcaaaacaaaacttaaatttcatgtcttagaaaaacatcgaccacacaatcaaataaataacattgataagagccttctggggcagcggcgcacggaggcgagtccacagcagtcactctcccggcccttctttggaagccctgctctgactgtgtctctgtgggtcgccgcgtgggccggcgtgaccccccgggggcacagggctggcagtggctggctccagcggcgtccacgaggacagagactcgtgcaccgtcagggcgtgctcctccatctggcgctgcaggctgtccatctcctgcttgagctgctggaggcagctgttcaggttcttgaggggctccttgctcacggcgggcggtggtctcagcagctcctccagcagcgaggcgggaactgggcagtccgggatcttgatgggcgtggcagggttggaagagctggcctcgcctttcggctcctttctcgtcttggccgcgccgcggcgtaggtccagcttgagctgctggttctgctggagcagggtcttcatgttgttcttcagctccgacacttttgcctggagcataaatttatccttctgggtcatggacaggtcttcctgggccatctccaactcagacttgacgttctgcagcagctgctgtagcccttccagttccttcctgccctgctgctccgtcaagtccagctgctgcttcaaggactggatttctctttctttctgatccacctcccatttgagattttccatctcttggtttcccacgggctgtttgctgagctgctcgtccagctgcttctgcaggagctggagctgtgcccgggcctcggccagctctgcttggaactgtgctatctcctgggaatgtttcccctcccgaatctgaaggtcgtcggcctcggcctgcagcttctgcaccaggtgttccttggcctgcagctccttcttcacctcactcagctccaaggaggccgccttgaagtggcggcggttatgcccggcttccaccttggcagcagccacctgctccttgaggctgttcaccttctccttctccttctctagtgaggcctgcagggcctggacaagatgcttcatctggcgatcctcctcttctttgcgctgcaaaactgcctgcacctgaaggttcaactggactaggtctgcctccctcttggccaaagctgtttctaggatgctgttgtgttcccgcagagctgcgttggactgaccgaggcccgtaagcttccctttctcgtgctctaattcaagagccaacttcttgtttgactcctcaaggcgttttatcttcttcctaaagcctctggattcttgaagctcgtcctccagctccagcaccttctcccgggactcctccagctcctggctggtcagcgctatgacctcctgcagttccttttccagcagcgtcttgctatgactgacagcctgcagctccgcctccagggcctggatcctttcatgtagagccaggctgctgtcactgctgccaccctgggctcggagctggcccagctccgcgtccgcagcctccttggccgcgagggcctcctgcaggcggcggctgaggatgcccacggcgttctcgtaggccttatgtttggtcttcatctccttctgggcgctggtcaagtctgagcccagccgcctcatcttctgcttctgttccgtgatggccttccgggcctcttgctgcaactcttcgatttgtttcttcagcgcctcattggcctctgtgaccgcgaccatctgctccttatcgaactgcaacgactgcaagtgtgtttccatctcgtctcgctccttctgcgccgactggagatgcccttcaaggtccgccatgtgctgacggacctgggccacctctctgtgcaggcgcgagagctccgcctcggcagtccgcttctccccgtgcacttgcatcagctcctgccgcagctccttcagctccgagtccagcctcttcctggtggctttcagctcactgatgagctggtctttggaggtggcgtcgcgccggtaggcctccaccatcaccttttgttggagaaactgttcctttattttttgcatttgctttttcagagcagcagtctcctgctgcaggtgttccacctggccggatttgatagctaattcttctcttaacttctctaaagtttccgacgtttcctcggtaccttcttccaagcgtcttgctcctctgtcaagctcctccttgccactcttggccgcctgcaaagccgcctccaagatgatcttctcgttctgcaggaggcagatcgtgtcctccctggaggcggcctcgccctgcagctcccccagcctggcctgcagctcatcgtagtgtgtctgcagggcatcgagggactgctccctgctctgcagagcctcctgagtcaaggtgagctgtttcatcaggtccaggtgctcctgctgcaaagcctcaagctgctggtctcgctggagtaaagtcaacttcacctgctccagctgctgctccagggatgccgccgagtccgccatcctctgcagccgctccctctcaccttcaaactcttccagcctcctctgaaggtcctcctccaccatcgtctttgcctcctgaatctgcatgaaggctgcttcctgatccaacatgtcagcctcaatgccctgcagctgtgccgcgatgcgccccttctccttcatggacctgtgctgagtttccgtcagctgctgggacagggacacattctcgagtttcaggtgctccaggagacctgcctgggtcatctgtccaacctggatgtgggccatctcaccctgcagcctgacgcgggcctcctgtgccagggcgagctgctgctggtaccactgccggacactctgcagggacgagatctccgcctgcgacgccttcagcttgctggtcagcgtcgtccgctccagctgcacctgctgaagctggctctgcaaggctgtcatctgctgtcgcaggtcgtgcactgtgttgtccttgctgagcatgctcctctgcatgtcctctaccttggccataagcctctggtactgctcctcggccacctgcaagtcgttgttggacgacgccaggctggcattttttgcctccagcatgttctgcaggtcagtcatggctcgctccaggtcccagcacgactgcttcagggtgtccacctccgagctcagcgaatcctgccgctgctggctgctgtggctgcactccacctgcgcctgcagcttcgtgctgagggcggccagctgggcctgcagctcagccttctctttaagtgcctgactcgcctccagtgacaaggcttccagctgtccttcgagtcgcattttctctttgagcacctgcagcatctcctcctgtgtttctgctgcagagctctccaaggacacgctgctgcagatgctgtctctccgactccgcacctccccgttgacctcctgcccctggtcttggtgctcagcggctgcggcctggaggacgtccttaatggaggggaactggcccagggtatccgcaggaatctcctggccgttgaccatatagggggtgtcctgcgtgcccactgtcttcgacagaatgccataggtccctcgggtggaggcgctgctgtacgatgagctgtcgctgtcatttccatccacctcagacacgctgtctccagccagggaggtgttctccagacggtcgtcagtgtcgggggacaggctgatctcagacacaacggacgccgcactgcttctgttctgcttcagggaacccttggtagaatcgggagccgggacatttcccccagaattccccgcatttgaatcttcagttctgtaatcggccagagaccggattttgcttgatttggaagtttttttctccctaggatgtgccggaagccccaggctgcccaccttaggcccccgagggacactggtgcgcaggaaggaatattcttttgtcatagccagggtactggcccttggtaagttttctgggtttaacatgagctcaggatcaagcgtgctaaaaagtctcgttttggttgcaggttgactggacctctcctgctggcgcttcaccctgtactgtttgagctgctcttccagccacttccgagcctgaagtcggacctgctcctccttctccaggggcaggggagaatctgtagagcctggagaggcatcagggcccactgggcttgtggtgggatcgagagacgacggagggtctgggaagggtggcgttggcccgttctgacagaggcctccctggccaggtccatccgggctttccccttccgtggatgctctgtttacctcggcacactggactttgtcctgctggtcaggtggcaccagtgggcccgggggcttcagtggggcctcggggagagacgaggggccactgtgggatctgtcctcctggaggccatcttgctcggccgacgcgccgtccatggtcaggacgacaccagctgagctgacgctgaggggctacaagtgaaccttggacaagcttggcttctgccatcagcaacagccaagagctcctgggaggggccctactgtgtctcccattttcaggagaagatctgatgactcacaaatgacttgatgtcaaaccagctaatatcatgatacctccgactgtgatgaggccgccttcagaaagtgaccttaagagtttgcggacctttccctagtagaaacgcaacttccggaactgcaggaccaactctttcaggaagctgaac

SEQ ID NO: 14317 - RNA, 6293 nt, Homo sapiens
  source 1..6293: mol_type = other RNA
gctgggattacaggcatgagccaccgcgcccggcccgatttcttgattttaaaattaaaacaaaggggtagtacagccaaaataaataagaacgtaaattgccgtatttttttttctaatggtacaagaacaatttagtaaataacatcttcaacttaagataaaaagtaggatatatttataatgaaattttcaagtattatttcaaaattaaccctgtacaaatgatatattttggaaattccaatatttgctagagaatattttttaaataccaaacatctttgtggttaatgctaccttaaccttaccaattaaccttctaaaagtatattacaacagaacacaaatagcttaaaacacaccatactgttttctccacaaaacagacaccagacaccgacatgagcacatctggcctggccagtgactcagaacctcatttcagaccagtacatctgcagaggaggccacgcggacccattctctctctcctaactcatataataaatattattttagattttcttagcaaactaggggacaacttacagaccccacctctcccagtcagccagtgtctgcagggtttcaggatttggggtaggaaacagaagatctcacacatgtcgtgctgattttaaataaggcatctgtctctgagacacctgggagagcacagccaccttcctcacggtgcctgcctgtctcttccggaagtcgcctctgcttgccacatgatgctggtgtaaccacaaaagatccaggacttctcgatgactgcagaagtacaggtgctcctacacacgagtacaggcgctcccacagacaatggtaaagattttcacttggggaacaggagtgtgaggtttgttaccgcctgcgacctacacctggctgactccaggggaaaccgcgggagtcgctgcagggagcccctggtctgctctcctcctcctcctccaccggcctctccctgtgcccccccaaaggtcagatcagatatggggcctcagtgtccttgtgcctcctgatggccgtcaggcctgaccaagggtccaagctgccccttcccagtggccagccacggtggaatcacacagggccagtggcctgagaggaagagaccagcaggaaggaaagatcctcagcaacaaagtaaaaccagaacaacagaggacctttctgtgtaagaatatttggctttagaaggtaaataaaataattatatttcttagaattttctgactatccctaaatcctgcaggtaaattattcccaacaaattttcaaaaggcaatcaataataagtaggttcttcttcaataacatgagcatatgcttcttaaagactgggtgacaggccgggcgcaggggctcacgcctgtaatcccagcactttgggaggctgagatgggcagatcacttgaggtcaggagatcgagaccatcctggccaacatggtgaaaccccattgctactaaaaatacaaacattagcctggcatagtggcgcacgcctgtaatcccagctactcgagaggctgaggcaggagaatcgcatgaacctgggaggcggagcttgcagtgagcggagagtgtgccactgcactccagcctgggcaacaaagcgagactctgtctcaaaaaaaaaaaaaaaaaaaaaacaaagattggattatgatattcagtatctatgtacacatcctatggtgggatggctatccaaaaaaacaagtaaaaagccaaaggtacagataaaatttcatttctgcggaaaagtaaagctcttactgaatggaacagggaagtgagaaactgcagccggcctggccaggcgcggtgccgcagaccctgtcacacagctgctcccagttacgcagcctctccctgtcacccgcagagagcagcatcggtggccgctcagaagccacgacctacaagtaacccttcagacacgttcaaagctcctcgccgagagcctatcaggcttttaagagttggtcattccatgtgaaaagctaattgtgatcttcgaatgtttttctagtccttggctctcattctgctatatattttacttcttgttaaaggcaaaacaaaacttaaatttcatgtcttagaaaaacatcgaccacacaatcaaataaataacattgataagagccttctggggcagcggcgcacggaggcgagtccacagcagtcactctcccggcccttctttggaagccctgctctgactgtgtctctgtgggtcgccgcgtgggccggcgtgaccccccgggggcacagggctggcagtggctggctccagcggcgtccacgaggacagagactcgtgcaccgtcagggcgtgctcctccatctggcgctgcaggctgtccatctcctgcttgagctgctggaggcagctgttcaggttcttgaggggctccttgctcacggcgggcggtggtctcagcagctcctccagcagcgaggcgggaactgggcagtccgggatcttgatgggcgtggcagggttggaagagctggcctcgcctttcggctcctttctcgtcttggccgcgccgcggcgtaggtccagcttgagctgctggttctgctggagcagggtcttcatgttgttcttcagctccgacacttttgcctggagcataaatttatccttctgggtcatggacaggtcttcctgggccatctccaactcagacttgacgttctgcagcagctgctgtagcccttccagttccttcctgccctgctgctccgtcaagtccagctgctgcttcaaggactggatttctctttctttctgatccacctcccatttgagattttccatctcttggtttcccacgggctgtttgctgagctgctcgtccagctgcttctgcaggagctggagctgtgcccgggcctcggccagctctgcttggaactgtgctatctcctgggaatgtttcccctcccgaatctgaaggtcgtcggcctcggcctgcagcttctgcaccaggtgttccttggcctgcagctccttcttcacctcactcagctccaaggaggccgccttgaagtggcggcggttatgcccggcttccaccttggcagcagccacctgctccttgaggctgttcaccttctccttctccttctctagtgaggcctgcagggcctggacaagatgcttcatctggcgatcctcctcttctttgcgctgcaaaactgcctgcacctgaaggttcaactggactaggtctgcctccctcttggccaaagctgtttctaggatgctgttgtgttcccgcagagctgcgttggactgaccgaggcccgtaagcttccctttctcgtgctctaattcaagagccaacttcttgtttgactcctcaaggcgttttatcttcttcctaaagcctctggattcttgaagctcgtcctccagctccagcaccttctcccgggactcctccagctcctggctggtcagcgctatgacctcctgcagttccttttccagcagcgtcttgctatgactgacagcctgcagctccgcctccagggcctggatcctttcatgtagagccaggctgctgtcactgctgccaccctgggctcggagctggcccagctccgcgtccgcagcctccttggccgcgagggcctcctgcaggcggcggctgaggatgcccacggcgttctcgtaggccttatgtttggtcttcatctccttctgggcgctggtcaagtctgagcccagccgcctcatcttctgcttctgttccgtgatggccttccgggcctcttgctgcaactcttcgatttgtttcttcagcgcctcattggcctctgtgaccgcgaccatctgctccttatcgaactgcaacgactgcaagtgtgtttccatctcgtctcgctccttctgcgccgactggagatgcccttcaaggtccgccatgtgctgacggacctgggccacctctctgtgcaggcgcgagagctccgcctcggcagtccgcttctccccgtgcacttgcatcagctcctgccgcagctccttcagctccgagtccagcctcttcctggtggctttcagctcactgatgagctggtctttggaggtggcgtcgcgccggtaggcctccaccatcaccttttgttggagaaactgttcctttattttttgcatttgctttttcagagcagcagtctcctgctgcaggtgttccacctggccggatttgatagctaattcttctcttaacttctctaaagtttccgacgtttcctcggtaccttcttccaagcgtcttgctcctctgtcaagctcctccttgccactcttggccgcctgcaaagccgcctccaagatgatcttctcgttctgcaggaggcagatcgtgtcctccctggaggcggcctcgccctgcagctcccccagcctggcctgcagctcatcgtagtgtgtctgcagggcatcgagggactgctccctgctctgcagagcctcctgagtcaaggtgagctgtttcatcaggtccaggtgctcctgctgcaaagcctcaagctgctggtctcgctggagtaaagtcaacttcacctgctccagctgctgctccagggatgccgccgagtccgccatcctctgcagccgctccctctcaccttcaaactcttccagcctcctctgaaggtcctcctccaccatcgtctttgcctcctgaatctgcatgaaggctgcttcctgatccaacatgtcagcctcaatgccctgcagctgtgccgcgatgcgccccttctccttcatggacctgtgctgagtttccgtcagctgctgggacagggacacattctcgagtttcaggtgctccaggagacctgcctgggtcatctgtccaacctggatgtgggccatctcaccctgcagcctgacgcgggcctcctgtgccagggcgagctgctgctggtaccactgccggacactctgcagggacgagatctccgcctgcgacgccttcagcttgctggtcagcgtcgtccgctccagctgcacctgctgaagctggctctgcaaggctgtcatctgctgtcgcaggtcgtgcactgtgttgtccttgctgagcatgctcctctgcatgtcctctaccttggccataagcctctggtactgctcctcggccacctgcaagtcgttgttggacgacgccaggctggcattttttgcctccagcatgttctgcaggtcagtcatggctcgctccaggtcccagcacgactgcttcagggtgtccacctccgagctcagcgaatcctgccgctgctggctgctgtggctgcactccacctgcgcctgcagcttcgtgctgagggcggccagctgggcctgcagctcagccttctctttaagtgcctgactcgcctccagtgacaaggcttccagctgtccttcgagtcgcattttctctttgagcacctgcagcatctcctcctgtgtttctgctgcagagctctccaaggacacgctgctgcagatgctgtctctccgactccgcacctccccgttgacctcctgcccctggtcttggtgctcagcggctgcggcctggaggacgtccttaatggaggggaactggcccagggtatccgcaggaatctcctggccgttgaccatatagggggtgtcctgcgtgcccactgtcttcgacagaatgccataggtccctcgggtggaggcgctgctgtacgatgagctgtcgctgtcatttccatccacctcagacacgctgtctccagccagggaggtgttctccagacggtcgtcagtgtcgggggacaggctgatctcagacacaacggacgccgcactgcttctgttctgcttcagggaacccttggtagaatcgggagccgggacatttcccccagaattccccgcatttgaatcttcagttctgtaatcggccagagaccggattttgcttgatttggaagtttttttctccctaggatgtgccggaagccccaggctgcccaccttaggcccccgagggacactggtgcgcaggaaggaatattcttttgtcatagccagggtactggcccttggtaagttttctgggtttaacatgagctcaggatcaagcgtgctaaaaagtctcgttttggttgcaggttgactggacttaaaggtataagaagaacacgctggtcattttattgatcttcttctactgaagagatccttttgaaacatgacataggctgggcgcgatggtgggtgcctgtagtccc

SEQ ID NO: 14318 - RNA, 4866 nt, Homo sapiens
  source 1..4866: mol_type = other RNA
gctgggattacaggcatgagccaccgcgcccggcccgatttcttgattttaaaattaaaacaaaggggtagtacagccaaaataaataagaacgtaaattgccgtatttttttttctaatggtacaagaacaatttagtaaataacatcttcaacttaagataaaaagtaggatatatttataatgaaattttcaagtattatttcaaaattaaccctgtacaaatgatatattttggaaattccaatatttgctagagaatattttttaaataccaaacatctttgtggttaatgctaccttaaccttaccaattaaccttctaaaagtatattacaacagaacacaaatagcttaaaacacaccatactgttttctccacaaaacagacaccagacaccgacatgagcacatctggcctggccagtgactcagaacctcatttcagaccagtacatctgcagaggaggccacgcggacccattctctctctcctaactcatataataaatattattttagattttcttagcaaactaggggacaacttacagaccccacctctcccagtcagccagtgtctgcagggtttcaggatttggggtaggaaacagaagatctcacacatgtcgtgctgattttaaataaggcatctgtctctgagacacctgggagagcacagccaccttcctcacggtgcctgcctgtctcttccggaagtcgcctctgcttgccacatgatgctggtgtaaccacaaaagatccaggacttctcgatgactgcagaagtacaggtgctcctacacacgagtacaggcgctcccacagacaatggtaaagattttcacttggggaacaggagtgtgaggtttgttaccgcctgcgacctacacctggctgactccaggggaaaccgcgggagtcgctgcagggagcccctggtctgctctcctcctcctcctccaccggcctctccctgtgcccccccaaaggtcagatcagatatggggcctcagtgtccttgtgcctcctgatggccgtcaggcctgaccaagggtccaagctgccccttcccagtggccagccacggtggaatcacacagggccagtggcctgagaggaagagaccagcaggaaggaaagatcctcagcaacaaagtaaaaccagaacaacagaggacctttctgtgtaagaatatttggctttagaaggtaaataaaataattatatttcttagaattttctgactatccctaaatcctgcaggtaaattattcccaacaaattttcaaaaggcaatcaataataagtaggttcttcttcaataacatgagcatatgcttcttaaagactgggtgacaggccgggcgcaggggctcacgcctgtaatcccagcactttgggaggctgagatgggcagatcacttgaggtcaggagatcgagaccatcctggccaacatggtgaaaccccattgctactaaaaatacaaacattagcctggcatagtggcgcacgcctgtaatcccagctactcgagaggctgaggcaggagaatcgcatgaacctgggaggcggagcttgcagtgagcggagagtgtgccactgcactccagcctgggcaacaaagcgagactctgtctcaaaaaaaaaaaaaaaaaaaaaacaaagattggattatgatattcagtatctatgtacacatcctatggtgggatggctatccaaaaaaacaagtaaaaagccaaaggtacagataaaatttcatttctgcggaaaagtaaagctcttactgaatggaacagggaagtgagaaactgcagccggcctggccaggcgcggtgccgcagaccctgtcacacagctgctcccagttacgcagcctctccctgtcacccgcagagagcagcatcggtggccgctcagaagccacgacctacaagtaacccttcagacacgttcaaagctcctcgccgagagcctatcaggcttttaagagttggtcattccatgtgaaaagctaattgtgatcttcgaatgtttttctagtccttggctctcattctgctatatattttacttcttgttaaaggcaaaacaaaacttaaatttcatgtcttagaaaaacatcgaccacacaatcaaataaataacattgataagagccttctggggcagcggcgcacggaggcgagtccacagcagtcactctcccggcccttctttggaagccctgctctgactgtgtctctgtgggtcgccgcgtgggccggcgtgaccccccgggggcacagggctggcagtggctggctccagcggcgtccacgaggacagagactcgtgcaccgtcagggcgtgctcctccatctggcgctgcaggctgtccatctcctgcttgagctgctggaggcagctgttcaggttcttgaggggctccttgctcacggcgggcggtggtctcagcagctcctccagcagcgaggcgggaactgggcagtccgggatcttgatgggcgtggcagggttggaagagctggcctcgcctttcggctcctttctcgtcttggccgcgccgcggcgtaggtccagcttgagctgctggttctgctggagcagggtcttcatgttgttcttcagctccgacacttttgcctggagcataaatttatccttctgggtcatggacaggtcttcctgggccatctccaactcagacttgacgttctgcagcagctgctgtagcccttccagttccttcctgccctgctgctccgtcaagtccagctgctgcttcaaggactggatttctctttctttctgatccacctcccatttgagattttccatctcttggtttcccacgggctgtttgctgagctgctcgtccagctgcttctgcaggagctggagctgtgcccgggcctcggccagctctgcttggaactgtgctatctcctgggaatgtttcccctcccgaatctgaaggtcgtcggcctcggcctgcagcttctgcaccaggtgttccttggcctgcagctccttcttcacctcactcagctccaaggaggccgccttgaagtggcggcggttatgcccggcttccaccttggcagcagccacctgctccttgaggctgttcaccttctccttctccttctctagtgaggcctgcagggcctggacaagatgcttcatctggcgatcctcctcttctttgcgctgcaaaactgcctgcacctgaaggttcaactggactaggtctgcctccctcttggccaaagctgtttctaggatgctgttgtgttcccgcagagctgcgttggactgaccgaggcccgtaagcttccctttctcgtgctctaattcaagagccaacttcttgtttgactcctcaaggcgttttatcttcttcctaaagcctctggattcttgaagctcgtcctccagctccagcaccttctcccgggactcctccagctcctggctggtcagcgctatgacctcctgcagttccttttccagcagcgtcttgctatgactgacagcctgcagctccgcctccagggcctggatcctttcatgtagagccaggctgctgtcactgctgccaccctgggctcggagctggcccagctccgcgtccgcagcctccttggccgcgagggcctcctgcaggcggcggctgaggatgcccacggcgttctcgtaggccttatgtttggtcttcatctccttctgggcgctggtcaagtctgagcccagccgcctcatcttctgcttctgttccgtgatggccttccgggcctcttgctgcaactcttcgatttgtttcttcagcgcctcattggcctctgtgaccgcgaccatctgctccttatcgaactgcaacgactgcaagtgtgtttccatctcgtctcgctccttctgcgccgactggagatgcccttcaaggtccgccatgtgctgacggacctgggccacctctctgtgcaggcgcgagagctccgcctcggcagtccgcttctccccgtgcacttgcatcagctcctgccgcagctccttcagctccgagtccagcctcttcctggtggctttcagctcactgatgagctggtctttggaggtggcgtcgcgccggtaggcctccaccatcaccttttgttggagaaactgttcctttattttttgcatttgctttttcagagcagcagtctcctgctgcaggtgttccacctggccggatttgatagctaattcttctcttaacttctctaaagtttccgacgtttcctcggtaccttcttccaagcgtcttgctcctctgtcaagctcctccttgccactcttggccgcctgcaaagccgcctccaagatgatcttctcgttctgcaggaggcagatcgtgtcctccctggaggcggcctcgccctgcagctcccccagcctggcctgcagctcatcgtagtgtgtctgcagggcatcgagggactgctccctgctctgcagagcctcctgagtcaaggtgagctgtttcatcaggtccaggtgctcctgctgcaaagcctcaagctgctggtctcgctggagtaaagtcaacttcacctgctccagctgctgctccagggatgccgccgagtccgccatcctctgcagccgctccctctcaccttcaaactcttccagcctcctctgaaggtcctcctccaccatcgtctttgcctcctgaatctgcatgaaggctgcttcctgatccaacatgtcagcctgagcccaggaaactcaatgccctgcagctgtgccgcgatgcgccccttctccttcatggacctgtgctgagtttccgtcagctgctgggacagggacaca

SEQ ID NO: 14319 - RNA, 2856 nt, Homo sapiens
  source 1..2856: mol_type = other RNA
gctgggattacaggcatgagccaccgcgcccggcccttggggtgttttttatcttttaacacgggggacaccagaaggaaggaccacaggccccatgtctcatatagtgctgcctaagggcaaaaacacaagattgatactctccactctgaactgagagttagctgagccaatcatggagagactgaggcctggctcaggttccataggaccatgagctgctcagtggcaaggctgataaagccaatcctgagtacttactgagtgcccataaaagcttgcaggagaatttattgcatgagtaaatgaatggattttttttgtttatttgtgttttgtttttttgagacagagtctcactcttgtcacccaggctggagtgcagtggtgcgatctcggctcactgcaatctcagcctcctgggttcaagctgttcttctgtctcagccttctgagtagctgggattacaggcgcctgccaccacgcctgactaatttttatatttttagtagagacggggtttcaccatgttggccaggctggtctcgaactcctgacctcaggtgatctgcccgcctcagcctcccacagtgctgggattacaggcatgagccatcgcgcccagctgaatggatgttttatatgaccaaagctcttaaagctttccctgcagctccatgagctatggaaagaagaatctagaaagaagcccatgtgtaaggtatcaggtttgatataaatgggggtcactagatcttattctcagaccctcccaggctgaaggaggcccaccctagtccagcatctggagagcaaagctgccggggcagcacagacactgccctctttacacctcgctaatgtccaggagtccgcacttgtatgggaccaactcccaagagtacctgagagttctccctgtctggccctgttccaagacataaagatcaggagaaactgatttgtgtgtggacaaaaatagagaagcaagaaaaattcaatgtaactaaagctacccaccacctgacagccatctagaatgtacctgagccctgtgccagccatgaccacctctgtcatctcagcctcactgtcctgacacccccactgctagctagatcagagagagatgcagagagggccgggccccagggctttgagtctctctcctaagtgcaatcgatgaagcaggaggaatccaggctctgcctgccctggcagcagggtgcctcttcctagtctgtaggaggagggtttccccgaagaggccgaggcagagggagaggaggggaagagtctgtcagagaagaaccacaggagaggttgaccacggcagccttgagctcaaagagggacctcaagtcctaggcacagtggggtttttagtcactcacaaggggattgcggtcatcttgttgactctgacccttgagtttcttcttaaagatggaaattgaagtggaaggcttgtaaaaaatgctccagatttcccccgaagtccctggttgatgacaatccctaaggtcccctgaagcaggaacacgatgggatttgaatgtgacgtgcagaagtatctttgctacaatggctgtgactgtgaggatgaggagagttgccagaccatagactgtccatcctgggacagtctgaggtgggtggctggggctggtggtgatgacatagaggactttggaggaccgggcagcgctgacactgaggttggcctgctccgtgatcacctcggccaccgtctggttgacagcgggcctctcctgtggcagttcttccttgacggcttggtataaaacagcaaatccctgggcctgattgatgcgatcagagaagaaatacaagatgacgaagtccagagagacgttgaaggacagaggtgggcggctcctcccgtggaagcgggctaggacacggtgggtgtagccatccagaagctccaccatgtccgccgagtccctgatgtcaaatagggggaagctgaagtggatgtgggaggcccccggaacccggatggtccagtagcagaccctccccgtggcataggtgtcggggaagtcaggggaatagaccacagaagacatggctgagtagttcccaccgcaggcgcccacgagagtatcaaagaggatgatcctgccatcgccaccacagggttgggtgtgatccccgaagcagacgctgttgcattcggtactggctgcctccccgtacttccagtaatcaggattgtttccacagaagcaagcatagcctgactccatcccagcaaacttgaacctctgactccgacaaaaactgatgcaagtttgtatggtgagtttgttggacgttttactggtgccagttagaggaggtgggtttccatgatccttgtagcagccaaggtttccaggcatctggcaagcaggtatctcacagtacttccagtagacaccatcctcgtgctctgccacatagcaccaggggctcacgtctccatctggatttctgcaatagttgtgctcacccaggcccccctccccgttggggtatttcagagtgttgtatggatgctggaaagtctcgttccaaaacagacatggcttcccgccttgtagtgctgtccagttctgtgttcccctataatccgcaccattggctgtgaaacactcgggtccggggccgaggccggggctaggcgcgggccgggccgccagcgtgagcgccgcggcggagagcagggcgaggcgggcggctggcggcgccatgggccgtcagtgcggggccccggggcgcggcccggggtaaagggggcagcgcggggagccgggggcggccatgggagcaggacgcggggcccgagt

SEQ ID NO: 14320 - RNA, 2496 nt, Homo sapiens
  source 1..2496: mol_type = other RNA
gctgggattacaggcatgagccaccgcgcccggcccttggggtgttttttatcttttaacacgggggacaccagaaggaaggaccacaggccccatgtctcatatagtgctgcctaagggcaaaaacacaagattgatactctccactctgaactgagagttagctgagccaatcatggagagactgaggcctggctcaggttccataggaccatgagctgctcagtggcaaggctgataaagccaatcctgagtacttactgagtgcccataaaagcttgcaggagaatttattgcatgagtaaatgaatggattttttttgtttatttgtgttttgtttttttgagacagagtctcactcttgtcacccaggctggagtgcagtggtgcgatctcggctcactgcaatctcagcctcctgggttcaagctgttcttctgtctcagccttctgagtagctgggattacaggcgcctgccaccacgcctgactaatttttatatttttagtagagacggggtttcaccatgttggccaggctggtctcgaactcctgacctcaggtgatctgcccgcctcagcctcccacagtgctgggattacaggcatgagccatcgcgcccagctgaatggatgttttatatgaccaaagctcttaaagctttccctgcagctccatgagctatggaaagaagaatctagaaagaagcccatgtgtaaggtatcaggtttgatataaatgggggtcactagatcttattctcagaccctcccaggctgaaggaggcccaccctagtccagcatctggagagcaaagctgccggggcagcacagacactgccctctttacacctcgctaatgtccaggagtccgcacttgtatgggaccaactcccaagagtacctgagagttctccctgtctggccctgttccaagacataaagatcaggagaaactgatttgtgtgtggacaaaaatagagaagcaagaaaaattcaatgtaactaaagctacccaccacctgacagccatctagaatgtacctgagccctgtgccagccatgaccacctctgtcatctcagcctcactgtcctgacacccccactgctagctagatcagagagagatgcagagagggccgggccccagggctttgagtctctctcctaagtgcaatcgatgaagcaggaggaatccaggctctgcctgccctggcagcagggtgcctcttcctagtctgtaggaggagggtttccccgaagaggccgaggcagagggagaggaggggaagagtctgtcagagaagaaccacaggagaggttgaccacggcagccttgagctcaaagagggacctcaagtcctaggcacagtggggtttttagtcactcacaaggggattgcggtcatcttgttgactctgacccttgagtttcttcttaaagatggaaattgaagtggaaggcttgtaaaaaatgctccagatttcccccgaagtccctggttgatgacaatccctaaggtcccctgaagcaggaacacgatgggatttgaatgtgacgtgcagaagtatctttgctacaatggctgtgactgtgaggatgaggagagttgccagaccatagactgtccatcctgggacagtctgaggtgggtggctggggctggtggtgatgacatagaggactttggaggaccgggcagcgctgacactgaggttggcctgctccgtgatcacctcggccaccgtctggttgacagcgggcctctcctgtggcagttcttccttgacggcttggtataaaacagcaaatccctgggcctgattgatgcgatcagagaagaaatacaagatgacgaagtccagagagacgttgaaggacagaggtgggcggctcctcccgtggaagcgggctaggacacggtgggtgtagccatccagaagctccaccatgtccgccgagtccctgatgtcaaatagggggaagctgaagtggatgtgggaggcccccggaacccggatggtccagtagcagaccctccccgtggcataggtgtcggggaagtcaggggaatagaccacagaagacatggctgagtagttcccaccgcaggcgcccacgagagtctggcaagcaggtatctcacagtacttccagtagacaccatcctcgtgctctgccacatagcaccaggggctcacgtctccatctggatttctgcaatagttgtgctcacccaggcccccctccccgttggggtatttcagagtgttgtatggatgctggaaagtctcgttccaaaacagacatggcttcccgccttgtagtgctgtccagttctgtgttcccctataatccgcaccattggctgtgaaacactcgggtccggggccgaggccggggctaggcgcgggccgggccgccagcgtgagcgccgcggcggagagcagggcgaggcgggcggctggcggcgccatgggccgtcagtgcgg

SEQ ID NO: 14321 - RNA, 4234 nt, Homo sapiens
  source 1..4234: mol_type = other RNA
gctgggattacaggcatgagccaccgcgcccggcccttggggtgttttttatcttttaacacgggggacaccagaaggaaggaccacaggccccatgtctcatatagtgctgcctaagggcaaaaacacaagattgatactctccactctgaactgagagttagctgagccaatcatggagagactgaggcctggctcaggttccataggaccatgagctgctcagtggcaaggctgataaagccaatcctgagtacttactgagtgcccataaaagcttgcaggagaatttattgcatgagtaaatgaatggattttttttgtttatttgtgttttgtttttttgagacagagtctcactcttgtcacccaggctggagtgcagtggtgcgatctcggctcactgcaatctcagcctcctgggttcaagctgttcttctgtctcagccttctgagtagctgggattacaggcgcctgccaccacgcctgactaatttttatatttttagtagagacggggtttcaccatgttggccaggctggtctcgaactcctgacctcaggtgatctgcccgcctcagcctcccacagtgctgggattacaggcatgagccatcgcgcccagctgaatggatgttttatatgaccaaagctcttaaagctttccctgcagctccatgagctatggaaagaagaatctagaaagaagcccatgtgtaaggtatcaggtttgatataaatgggggtcactagatcttattctcagaccctcccaggctgaaggaggcccaccctagtccagcatctggagagcaaagctgccggggcagcacagacactgccctctttacacctcgctaatgtccaggagtccgcacttgtatgggaccaactcccaagagtacctgagagttctccctgtctggccctgttccaagacataaagatcaggagaaactgatttgtgtgtggacaaaaatagagaagcaagaaaaattcaatgtaactaaagctacccaccacctgacagccatctagaatgtacctgagccctgtgccagccatgaccacctctgtcatctcagcctcactgtcctgacacccccactgctagctagatcagagagagatgcagagagggccgggccccagggctttgagtctctctcctaagtgcaatcgatgaagcaggaggaatccaggctctgcctgccctggcagcagggtgcctcttcctagtctgtaggaggagggtttccccgaagaggccgaggcagagggagaggaggggaagagtctgtcagagaagaaccacaggagaggttgaccacggcagccttgagctcaaagagggacctcaagtcctaggcacagtggggtttttagtcactcacaaggggattgcggtcatcttgttgactctgacccttgagtttcttcttaaagatggaaattgaagtggaaggcttgtaaaaaatgctccagatttcccccgaagtccctggttgatgacaatccctaaggtcccctgaagcaggaacacgatgggatttgaatgtgacgtgcagaagtatctttgctacaatggctgtgactgtgaggatgaggagagttgccagaccatagactgtccatccttcaactctgtggcttccagcccccatgggtggcgcccaggaattgctacctgggacagtctgaggtgggtggctggggctggtggtgatgacatagaggactttggaggaccgggcagcgctgacactgaggttggcctgctccgtgatcacctcggccaccgtctggttgacagcgggcctctcctgtggcagttcttccttgacggcttggtataaaacagcaaatccctgggcctgattgatgcgatcagagaagaaatacaagatgacgaagtccagagagacgttgaaggacagaggtgggcggctcctcccgtggaagcgggctaggacacggtgggtgtagccatccagaagctccaccatgtccgccgagtccctgatgtcaaatagggggaagctgaagtggatgtgggaggcccccggaacccggatggtccagtagcagaccctccccgtggcataggtgtcggggaagtcaggggaatagaccacagaagacatggctgagtagttcccaccgcaggcgcccacgagagtatcaaagaggatgatcctgccatcgccaccacagggttgggtgtgatccccgaagcagacgctgttgcattcggtactggctgcctccccgtacttccagtaatcaggattgtttccacagaagcaagcatagcctgactccatcccagcaaacttgaacctctgactccgacaaaaactgatgcaagtttgtatggtgagtttgttggacgttttactggtgccagttagaggaggtgggtttccatgatccttgtagcagccaaggtttccaggcactccgagttgttcttttaacagtaagttctgatccatgctctgcaggtcaagagcagttcagatttccctctgctcccatttgagttgtacttcaggtctgcctcctgcttgttgtagctctacacataacacaccaaggggcagagatctggtttccacacaatggcccaccattcagccagattctgctttgtccctaaacattcattccccctggctcctgctgggtctgttatattcagatatgaactttccaggaatctgatcatgtcacaggactttttctgtatgacaagttcaatactaatcatgaatagcaggcttcatgcagaggtttagtattattcatgaaaattgtgactccacatccagaaatagggcaaaagtggcctaaaataggatggctgtatctctgttaaatccaccaggcaattacaaacatctcttgctacaaactgtaaaacaggttttgctcaactatgttaatcagacacactagaagtacaatatgctgccagactcaatgtctgaggtccggcttgatggggagccctggtccccacagggtaaactgaagggttttccaaagaaccaaagccagacaccacccaccctctatccccagaaaccaggtactatagagctctcattcccaacttctacaaatctctctgcccagaccatctcaaggctagctttagagattttagagggttatcaaggggccacagaaaaactgaaataatatttaattttccttttttggaacaggaaagcatatccggtaaatattacaaattagaggcatactaagcggtttatagcattttgttataattctttcttctggaacctggtttcaatgaccacatgaatcagtccctattggcccagactgtattttagaaatgcaagtcaaagattatctttccaaataaaagtgcccagattgaaaccccctctttaccactcccaagagaatgacacaggctggtactaaaagactatctttgtgttgaacaaatggaccgaggaaaatctgctttcctctccctctgcttctttcttctttacataactagaggcaaatgagatgtttttcattttaaaaatttgattaagcagactgagcaaaagcccattcttctggtctttactgttttctaagtttggggactggatgaaggcacactcaggttggaaggatagtgaagctaagcaaaaggtgagtactaggtctgcagcactggtcaggggctgcctttccccctggaggcctcagcattcagatgctattccaggtatcagtgaaagggttgccagatcccatacacaagactcctgacctgagaggtgagaaagagggcaatgcaaagagcaggtttaaataataagaaaaaaataacccagataggatgttacgaattcactgtctttttcctcagctctaggcactgagctcttctggcatattttaaaatacattatatatactacattaatagactccttatagaagcagatcttgctttagtttctgtggttcaaaccttctgcaagacctttctacacacagtattttctttaccttgtttaaaagtatagtcatgtatctcttaggcaaggtttcgctctgagaactgcattgtcatataattttgttgttgtgtgaccatcatagagtgcacttgcacaaactgagatgtgatagtctactacacacctagtctataatgggatagcctgtcactcctaggctacaaacctgagcagc

SEQ ID NO: 14322 - RNA, 2824 nt, Homo sapiens
  source 1..2824: mol_type = other RNA
gctgggattacaggcatgagccaccgcgcccggcccttggggtgttttttatcttttaacacgggggacaccagaaggaaggaccacaggccccatgtctcatatagtgctgcctaagggcaaaaacacaagattgatactctccactctgaactgagagttagctgagccaatcatggagagactgaggcctggctcaggttccataggaccatgagctgctcagtggcaaggctgataaagccaatcctgagtacttactgagtgcccataaaagcttgcaggagaatttattgcatgagtaaatgaatggattttttttgtttatttgtgttttgtttttttgagacagagtctcactcttgtcacccaggctggagtgcagtggtgcgatctcggctcactgcaatctcagcctcctgggttcaagctgttcttctgtctcagccttctgagtagctgggattacaggcgcctgccaccacgcctgactaatttttatatttttagtagagacggggtttcaccatgttggccaggctggtctcgaactcctgacctcaggtgatctgcccgcctcagcctcccacagtgctgggattacaggcatgagccatcgcgcccagctgaatggatgttttatatgaccaaagctcttaaagctttccctgcagctccatgagctatggaaagaagaatctagaaagaagcccatgtgtaaggtatcaggtttgatataaatgggggtcactagatcttattctcagaccctcccaggctgaaggaggcccaccctagtccagcatctggagagcaaagctgccggggcagcacagacactgccctctttacacctcgctaatgtccaggagtccgcacttgtatgggaccaactcccaagagtacctgagagttctccctgtctggccctgttccaagacataaagatcaggagaaactgatttgtgtgtggacaaaaatagagaagcaagaaaaattcaatgtaactaaagctacccaccacctgacagccatctagaatgtacctgagccctgtgccagccatgaccacctctgtcatctcagcctcactgtcctgacacccccactgctagctagatcagagagagatgcagagagggccgggccccagggctttgagtctctctcctaagtgcaatcgatgaagcaggaggaatccaggctctgcctgccctggcagcagggtgcctcttcctagtctgtaggaggagggtttccccgaagaggccgaggcagagggagaggaggggaagagtctgtcagagaagaaccacaggagaggttgaccacggcagccttgagctcaaagagggacctcaagtcctaggcacagtggggtttttagtcactcacaaggggattgcggtcatcttgttgactctgacccttgagtttcttcttaaagatggaaattgaagtggaaggcttgtaaaaaatgctccagatttcccccgaagtccctggttgatgacaatccctaaggtcccctgaagcaggaacacgatgggatttgaatgtgacgtgcagaagtatctttgctacaatggctgtgactgtgaggatgaggagagttgccagaccatagactgtccatccttcaactctgtggcttccagcccccatgggtggcgcccaggaattgctacctgggacagtctgaggtgggtggctggggctggtggtgatgacatagaggactttggaggaccgggcagcgctgacactgaggttggcctgctccgtgatcacctcggccaccgtctggttgacagcgggcctctcctgtggcagttcttccttgacggcttggtataaaacagcaaatccctgggcctgattgatgcgatcagagaagaaatacaagatgacgaagtccagagagacgttgaaggacagaggtgggcggctcctcccgtggaagcgggctaggacacggtgggtgtagccatccagaagctccaccatgtccgccgagtccctgatgtcaaatagggggaagctgaagtggatgtgggaggcccccggaacccggatggtccagtagcagaccctccccgtggcataggtgtcggggaagtcaggggaatagaccacagaagacatggctgagtagttcccaccgcaggcgcccacgagagtatcaaagaggatgatcctgccatcgccaccacagggttgggtgtgatccccgaagcagacgctgttgcattcggtactggctgcctccccgtacttccagtaatcaggattgtttccacagaagcaagcatagcctgactccatcccagcaaacttgaacctctgactccgacaaaaactgatgcaagtttgtatggtgagtttgttggacgttttactggtgccagttagaggaggtgggtttccatgatccttgtagcagccaaggtttccaggcatctggcaagcaggtatctcacagtacttccagtagacaccatcctcgtgctctgccacatagcaccaggggctcacgtctccatctggatttctgcaatagttgtgctcacccaggcccccctccccgttggggtatttcagagtgttgtatggatgctggaaagtctcgttccaaaacagacatggcttcccgccttgtagtgctgtccagttctgtgttcccctataatccgcaccattggctgtgaaacactcgggtccggggccgaggccggggctaggcgcgggccgggccgccagcgtgagcgccgcggcggagagcagggcgaggcgggcggctggcggcgccatgggccgtcagtgc

SEQ ID NO: 14323 - RNA, 2813 nt, Homo sapiens
  source 1..2813: mol_type = other RNA
gctgggattacaggcatgagccaccgcgcccggcccttggggtgttttttatcttttaacacgggggacaccagaaggaaggaccacaggccccatgtctcatatagtgctgcctaagggcaaaaacacaagattgatactctccactctgaactgagagttagctgagccaatcatggagagactgaggcctggctcaggttccataggaccatgagctgctcagtggcaaggctgataaagccaatcctgagtacttactgagtgcccataaaagcttgcaggagaatttattgcatgagtaaatgaatggattttttttgtttatttgtgttttgtttttttgagacagagtctcactcttgtcacccaggctggagtgcagtggtgcgatctcggctcactgcaatctcagcctcctgggttcaagctgttcttctgtctcagccttctgagtagctgggattacaggcgcctgccaccacgcctgactaatttttatatttttagtagagacggggtttcaccatgttggccaggctggtctcgaactcctgacctcaggtgatctgcccgcctcagcctcccacagtgctgggattacaggcatgagccatcgcgcccagctgaatggatgttttatatgaccaaagctcttaaagctttccctgcagctccatgagctatggaaagaagaatctagaaagaagcccatgtgtaaggtatcaggtttgatataaatgggggtcactagatcttattctcagaccctcccaggctgaaggaggcccaccctagtccagcatctggagagcaaagctgccggggcagcacagacactgccctctttacacctcgctaatgtccaggagtccgcacttgtatgggaccaactcccaagagtacctgagagttctccctgtctggccctgttccaagacataaagatcaggagaaactgatttgtgtgtggacaaaaatagagaagcaagaaaaattcaatgtaactaaagctacccaccacctgacagccatctagaatgtacctgagccctgtgccagccatgaccacctctgtcatctcagcctcactgtcctgacacccccactgctagctagatcagagagagatgcagagagggccgggccccagggctttgagtctctctcctaagtgcaatcgatgaagcaggaggaatccaggctctgcctgccctggcagcagggtgcctcttcctagtctgtaggaggagggtttccccgaagaggccgaggcagagggagaggaggggaagagtctgtcagagaagaaccacaggagaggttgaccacggcagccttgagctcaaagagggacctcaagtcctaggcacagtggggtttttagtcactcacaaggggattgcggtcatcttgttgactctgacccttgagtttcttcttaaagatggaaattgaagtggaaggcttgtaaaaaatgctccagatttcccccgaagtccctggttgatgacaatccctaaggtcccctgaagcaggaacacgatgggatttgaatgtgacgtgcagaagtatctttgctacaatggctgtgactgtgaggatgaggagagttgccagaccatagactgtccatccttcaactctgtggcttccagcccccatgggtggcgcccaggaattgctacctgggacagtctgaggtgggtggctggggctggtggtgatgacatagaggactttggaggaccgggcagcgctgacactgaggttggcctgctccgtgatcacctcggccaccgtctggttgacagcgggcctctcctgtggcagttcttccttgacggcttggtataaaacagcaaatccctgggcctgattgatgcgatcagagaagaaatacaagatgacgaagtccagagagacgttgaaggacagaggtgggcggctcctcccgtggaagcgggctaggacacggtgggtgtagccatccagaagctccaccatgtccgccgagtccctgatgtcaaatagggggaagctgaagtggatgtgggaggcccccggaacccggatggtccagtagcagaccctccccgtggcataggtgtcggggaagtcaggggaatagaccacagaagacatggctgagtagttcccaccgcaggcgcccacgagagtatcaaagaggatgatcctgccatcgccaccacagggttgggtgtgatccccgaagcagacgctgttgcattcggtactggctgcctccccgtacttccagtaatcaggattgtttccacagaagcaagcatagcctgactccatcccagcaaatctggcaagcaggtatctcacagtacttccagtagacaccatcctcgtgctctgccacatagcaccaggggctcacgtctccatctggatttctgcaatagttgtgctcacccaggcccccctccccgttggggtatttcagagtgttgtatggatgctggaaagtctcgttccaaaacagacatggcttcccgccttgtagtgctgtccagttctgtgttcccctataatccgcaccattggctgtgaaacactctgagtcatagggaagttcaaagcggcccagcggagagagagggcacgtcccgtccgtctgggtacaaggtcgtcccaggaccctaacctgcctctagcagggcgaacaagtccatcccgttcctcgcgaggcagaagttataatgtccgccaagcgggtgcagccgaggactcgggaaaaggggctgagcgccggctcctcccgcctccgctctgctctgcgc

SEQ ID NO: 14324 - RNA, 2547 nt, Homo sapiens
  source 1..2547: mol_type = other RNA
gctgggattacaggcatgagccaccgcgcccggcccttggggtgttttttatcttttaacacgggggacaccagaaggaaggaccacaggccccatgtctcatatagtgctgcctaagggcaaaaacacaagattgatactctccactctgaactgagagttagctgagccaatcatggagagactgaggcctggctcaggttccataggaccatgagctgctcagtggcaaggctgataaagccaatcctgagtacttactgagtgcccataaaagcttgcaggagaatttattgcatgagtaaatgaatggattttttttgtttatttgtgttttgtttttttgagacagagtctcactcttgtcacccaggctggagtgcagtggtgcgatctcggctcactgcaatctcagcctcctgggttcaagctgttcttctgtctcagccttctgagtagctgggattacaggcgcctgccaccacgcctgactaatttttatatttttagtagagacggggtttcaccatgttggccaggctggtctcgaactcctgacctcaggtgatctgcccgcctcagcctcccacagtgctgggattacaggcatgagccatcgcgcccagctgaatggatgttttatatgaccaaagctcttaaagctttccctgcagctccatgagctatggaaagaagaatctagaaagaagcccatgtgtaaggtatcaggtttgatataaatgggggtcactagatcttattctcagaccctcccaggctgaaggaggcccaccctagtccagcatctggagagcaaagctgccggggcagcacagacactgccctctttacacctcgctaatgtccaggagtccgcacttgtatgggaccaactcccaagagtacctgagagttctccctgtctggccctgttccaagacataaagatcaggagaaactgatttgtgtgtggacaaaaatagagaagcaagaaaaattcaatgtaactaaagctacccaccacctgacagccatctagaatgtacctgagccctgtgccagccatgaccacctctgtcatctcagcctcactgtcctgacacccccactgctagctagatcagagagagatgcagagagggccgggccccagggctttgagtctctctcctaagtgcaatcgatgaagcaggaggaatccaggctctgcctgccctggcagcagggtgcctcttcctagtctgtaggaggagggtttccccgaagaggccgaggcagagggagaggaggggaagagtctgtcagagaagaaccacaggagaggttgaccacggcagccttgagctcaaagagggacctcaagtcctaggcacagtggggtttttagtcactcacaaggggattgcggtcatcttgttgactctgacccttgagtttcttcttaaagatggaaattgaagtggaaggcttgtaaaaaatgctccagatttcccccgaagtccctggttgatgacaatccctaaggtcccctgaagcaggaacacgatgggatttgaatgtgacgtgcagaagtatctttgctacaatggctgtgactgtgaggatgaggagagttgccagaccatagactgtccatccttcaactctgtggcttccagcccccatgggtggcgcccaggaattgctacctgggacagtctgaggtgggtggctggggctggtggtgatgacatagaggactttggaggaccgggcagcgctgacactgaggttggcctgctccgtgatcacctcggccaccgtctggttgacagcgggcctctcctgtggcagttcttccttgacggcttggtataaaacagcaaatccctgggcctgattgatgcgatcagagaagaaatacaagatgacgaagtccagagagacgttgaaggacagaggtgggcggctcctcccgtggaagcgggctaggacacggtgggtgtagccatccagaagctccaccatgtccgccgagtccctgatgtcaaatagggggaagctgaagtggatgtgggaggcccccggaacccggatggtccagtagcagaccctccccgtggcataggtgtcggggaagtcaggggaatagaccacagaagacatggctgagtagttcccaccgcaggcgcccacgagagtctggcaagcaggtatctcacagtacttccagtagacaccatcctcgtgctctgccacatagcaccaggggctcacgtctccatctggatttctgcaatagttgtgctcacccaggcccccctccccgttggggtatttcagagtgttgtatggatgctggaaagtctcgttccaaaacagacatggcttcccgccttgtagtgctgtccagttctgtgttcccctataatccgcaccattggctgtgaaacactcgggtccggggccgaggccggggctaggcgcgggccgggccgccagcgtgagcgccgcggcggagagcagggcgaggcgggcggctggcggcgccatgggccgtcagtgcgg

SEQ ID NO: 14325 - RNA, 3018 nt, Homo sapiens
  source 1..3018: mol_type = other RNA
gctgggattacaggcatgagccaccgcgcccggccgagattgtttttttttaaaatgtgttgagttttgagagttcttcatggattctggatataagtcttttgtctgctatatggcttgcagatgttttcactcagtctgtagcatgtcttttcatcctcttaataggatccttcacagatcaagagtcccacattttgatgaagtccatgttataagtttttccacatatgaattgttattttggtgtcatgtctaagaactagatgttgaatatttctcctatgttttcttctaaaagttttatagtcttgcatgttacatttaaatctgtgaccctttggaactaattttgatattaggaggaatttcaggttgaggttcaaattttgcacatgaaaattccattattcccatagcatttgtggaaaaaatgccctttctctattgagttacttttgcacctttgtcagaaatcacttggccatatttgtgtagattcatttctgtactctgtattctgttccattggtctctgtgtccattccttcaataaaccacatgattgtgattactcttgcattaaagtaggacttaaaatactgtagcacagtattttcatctaaatgaaactaaattcatctttttaccttcacttttgcatataaatttaaaaatcagtttgtctatatagacaaaatatcctatgctaggattttgatggatttgtatttaagttacagatcaatctggggagaattgaaatttttactatgttgaatcttcccatccgtgaatatctcttcatttatttagaccttctttgattttgtttatagcactttttaagttttcagagtagacaatcttgtatacctaagaatttcatttttcagaagtattataaatgtaatttttgcaacatttaaaatttccagttatttattgctagcatgtaagtattgaatttagtattgcatgtgttgaccttgtattatttctgggttttcgtctcccccaagaaagtcaattttttacacaaggaagtcactctggttctccctccatgtttgtctacgcagtgtccacccttccaggtgtaggcaattcccttatctagagctcaaccccagcccttgggccttaacggtgtgtgtcctggggaggtggttcaagcatcccccgtcaatgtagagatgtggcagaaacccgttcacctgttatattggtatctggctccagaaagaaacgtttcattgctttgacataaaaataaattgatgaatgaagttaaacccagaagaagcttcgcaaagaggccgtgtaagcatctgcccatgggactcccttccacgcaccgtctttctcactaggtgttggggaggacagggagctggggctggggagggcagtgggaagagggagctttgcttagttacagggaaaggtgccccattcctgacagttgtaggactcttctttccctcctatcttccccctcaacctcttcaaatcgtagcctctggagaacctggactctggcggctgaggcctccctgggagtgaggtttgggcttccccgcctgcctttgcacagcagcctgtgtcaggtggcacctggacagcctgaggggagggacatcagcagaggggggacagggcggcagacacccccacatcccaccagctaggctgaggtggctgggacaacacccccagatggaacgagtactcttctcaccttcccaaatagatctttgagatgtcagcggctccaccacactggtcactgtaggtgagtgagctgaacacgtccctccatgaactgggaagagacacagagggagtcaaactatgcccttttcttgcctccattctcccagtcctctctgtgctgacatttgcctcagaggcagatcttgtttaaaaaacaaaattggcccaggctccatcagcaagtagtttcctcccttgggatttaaagaggtcttctgggaatcagcaggccccttttgtggcctctttgctgaattgtttctaaatatattttaattattctaggcctctagggacagagatgccgtcatcctcctttgccaccttttctatgatggtttgatgaggttaaaaaccccgacgaccagggttccactctatccttctcctaaacatttgttctatttctttgcctttaggagtggtgggtgtgtattgtcaggcctattgtaaaggatggtgtaaagtaaccatccaaaggttggttactttacacgtccctttggatgacttctgtacatagcactcttgctatgagtaattcctttgtagaaataggctctatggagaattgtctccttggacccttcatgtagctcacgacttttattatggaaataaatgaataaaagcctgcaattgtggacagacacaaatatgcttggacatggctatctctgatcttgtgtggctcaaaataacttacagagtcttcattttcagagtgttctcacccaaaaaggtaccaacttgggcatggaaagacctgtttctcctggactcctggacgtgccagccatcgagacagggaagacccactgatgtcttcaggatttgtccatcaccctggggactgtctggcctgctggcaggtgacagtggcctgtccaaaagtgtgagctacctgatgatgaaccagatgcaagggcaggactgtcttctgagagatgtctccccctcggtccttctgtcacttcagacattccaggtggaaggaggctctttgacctagtgaggcagagcggaggaaacccctctttggagattgccggatgtccctcttgtcctcctctgggagcatcagttgccgatttttgtcatcctggtaggagagcctttgtgacatttgatgcattctgatagtttctgttgtgctgtgctgcgctatgctattcttctaagggttagtcataaccgaccaaatggatgtcaccaccttctaatggatctagatccgcagct

SEQ ID NO: 14326 - RNA, 5122 nt, Homo sapiens
  source 1..5122: mol_type = other RNA
gctgggattacaggcatgagccaccgcgcccggccgtctttttttttttttcacttctctttagtcttttgataagctggtgaggtgcttttgcttgttccttaggaggggatttagtagatgctactttataagcttctttaactgtaaaatcctccttcattgtcaagtactagtaagcactggtgattccttgagatataatttcagaaatgttgggataaggcaccatgtctacatttcttggttaacaggcaaatgtggcacccagagggagtggcataatagccagttaccaataatatatcctgttaaaactcccaaagtactctgctttgtgttacagttgattattaagagtgcaactgttggctttttatgcctttgaaaaagtgcaatcatgtagaatgatgatcactagatggtgaatgactgactgaacagtgatattacgaatcccctatgtgcacaaaatagagaggtcaggtgtagacctatgacaaggaaccacagacatttagttatcaatgcattagttctgatggaactgacattattttcaaaaagaaataatttttaaaagggtcgatttctaactgtgtgagtatataaacacacactctatttcttcataactaacctgccttgatgctagcactaaatcatgacaggcacctggttgaaagtggttgcaagaagccatcaattttaagatgcattgtgatttccaaatagtaaaatatagccaggcgcagtgtctcacacctgtaatcccaacactttgggaggctgaggcaggtgcaggagttcaagatcagcctggaccaacatggcaaaaccccatctctactaaaaatacaagaattagccagtatggtggtgcacacctgtgtatccagctacttgggaggctgaggcacgagaatcacttgaacccgagaggtgcaggttgcagtgagccgaaatcacaccactgcactccagccttggtgacagaaagagagatcctgtcccaaaaaaaaaaaaaagtaaaatacataccatatgatcacacatttccaaagatcattgatcaaggctgaccaatcctattaggtatataatggatctttataacagacaactccagtagttaccataagtgatcaaacttggcactggtgatactgggggaaatggatactatctgcttctgaggtattgcaagatgaagtacacatcaccatctatgaagtgttctggtaaaaaatgtttaagcctctatttccaacttcatgttacgagaaatgtgaaggagaggcccatatcaaatttcaccatgaggaatgaaactaatgtgtgacattctataaaacagctttcctaaactcttcaaaagtctggattttttcaagtctcatttttttagctcagcttaagggataaactctgaattaaaatcccctcaaattctttatactgtactagatcttatccagaatgaactatctgaaattcaaatggatgagtggttatgggaagcttttctgaattcattcctcaaaacggttgtgcctctcctaagaattcaccagtagtaatactaataataaagacaatatgaacaatagctaatatgtattaagcataggctacataccagatactcttccaaggatatgatgcatactaaatccatctaatctctgtaacagcattattagttaccatcagcatttgaaacatcatgtccagaagagataagcattttgctcaccatcctacaggtagtatggaggtgaaatggtgatgacagtatggtatttgccatggataagggttttcctacatttgttacattaacagagttactctctaggatgaacttactgaagtttaacaaagactgaatagtgttggaaggcttctgcacatttaacatatctggtataaattatcttatgctgttacaggcattagaaaattttgattccctcatttgccaaatcttgctatagtatgaatattctgctattctaatcagagaggtgcaagtgaagaatttcttatttaaattgtcacttgtctcatgtcttgaaaagtgtgagtcttgtctcaaattatttctgggaaagaacaaactttgttttcaattctcaatcatttatggactgataattttgtaaaacagaatgttatggaaatgtcaaattgctataaaagttccaaatatttactcactttccacgtttatctcacaattgacagatgacaattttatgactgcaccagtctctggataataatttgggtagcatttgtctaaaggccttcctataattctaattcaaatgatttctcatttggatgaattctctgatgtactctaagatatttactgtgtctataagccttcccaaattccttatgtgcataggattacacagcagtatgaattctctgatgtgcagcaagaactgaattaagtttaggtccttcccacattcctcctatttaaactctttttaacaaataccaattatttgatgttaatcagaccttatgtcatgaatgaagatcttcacacattccttacatttaaatgattttacatcagtataaattgatatccaataagactgtacagaagtctaaaggccttttcatattaattatattcaaaatatttctcactagtatgaattgctggatagcaagataattgcccataaacagaaatgaatggcttttgcacaacccttacattcacaaggtttctcaagagtaagagttcttattatgataagttgtctatacacacacacaaaatattcttttacaactttcaatcataaggtttcatcagtatcaattttctcatttgagtaagttgtccacagaaaggcttccccacattcgttatatttgtagggtttatcattactatgagttctctcatgaacaagttttgagccacaagtaaaggtcttcccgaattccttacgttgataaagcttctcaccagtatgaaatctctgatgaacactaagttgatagccactaccaaaggccttcccacagtctttacattcataagacttctcattagtatggactctctcatgcttaactaggcttgaaccccaactgaaggccttcccacattccttacatttgaaaggtttctcaccggtatgaattttctgatgttgagtaaggtgatagccacgactaaaagccttcccacattctttacattcatagggtttctcccctgtatggattctttcatgttgaacaaggcttgatccacaattaaaagccttcccacattccttacattcatagggtttctcaccagtgtgaaatacctgatgtcgagtaagttgatacccactacaaaaggtctttccgcattctttacattcatgggatttctcaccagtatgaactctctcatgtttaacaaggcttgaaccccaactaaaggccttcccacattccttacattcaaaaggtttctcaccagtatggattttctgatgttgagaaaggtgatagccacgactaaaggcctttccacattctttacattcataaggtttctcaccagtatgaattctttcatgttgaataagacttgatccgcaattaaaagccttcccacattccttgcattcatagggtttctcaccagtatgaaatatctgatgtcgagtaagttgatagccccaacaaaaagcctttccacatattttacattcataaggtttcttaccagtatggattttctgatgctgagtaagctgatagccacgactgaaggccttcccacattctttacatttataaggtttctcacctgtatgaattatctcatgtttagcaaggcttgagccccaaaaaaaggccttcccacattccttacatttataagatttcacaccagtatgaattttctgatgttgggtaaggtgatagccacgactaaaggccttcccacattctttacattcatagggtttctcaccagtgtgaattctctcatgtttaacaaggcttgatccccagctaaaggtcttcccacattccttacactcatagggtttctcaccagtatgaaatctctgatgcacattgagttgataggcacttaaataattcttcccacattctttacattcaaagtgtttttcagctgtatgagttctctcatgttgaacaagttttgagccatgactgcaagccttcccacattccttacaaacataggatttctctgtattatgaattctttgatgtggagtaagagatttactttttctgtaagaaggtattttttcatagctgattatcatttgactgaagtatccctcttgatgtccttttagtccctcgaatatgcttttgcacttccaattatttctgaagatggatgcctcaaggccaagggttttacttttgtccttcatctcccactgggaaaaatttatttcaaaaatatcattttctgaaaatatttttttggtctcatacgtttttgactccaaatatcagtcatggttctggaattgcaagaactaattaatgctccatgggattcctctattggtgaagcacagaatccagaaaagccagaacagctctcgaacatcctgtagctgttattcaatgtaatgagacacattcactgtcaagattctcctgaaccttgatttctaaacatgcaaaaatccttttctcctcttcaaactccttcttagaaatctggcaacctggcagcacaccaaagagctcctagaggcccctcttctaggaatcccacctctagaacttccccatcaggtcttgacaagatcctgtcccgcggacacttccagatctaaaattctcatccttcttgcttgaaacgttcattatggggcttagcatagacttctttcttgcggtcatttaattgtggcaggcccgaagacaggctaaagggaaccatgcagagtccaagaaccttaaggacaccggaaaaggacccagagacctgtggttagtttggacccagaggctgatgggaaacaagagcctggaaatgctcgcaggctgggagaggagcttctggcaggcaagctcgccccgcccctaaaag

SEQ ID NO: 14327 - RNA, 4916 nt, Homo sapiens
  source 1..4916: mol_type = other RNA
gctgggattacaggcatgagccaccgcgcccggccgtctttttttttttttcacttctctttagtcttttgataagctggtgaggtgcttttgcttgttccttaggaggggatttagtagatgctactttataagcttctttaactgtaaaatcctccttcattgtcaagtactagtaagcactggtgattccttgagatataatttcagaaatgttgggataaggcaccatgtctacatttcttggttaacaggcaaatgtggcacccagagggagtggcataatagccagttaccaataatatatcctgttaaaactcccaaagtactctgctttgtgttacagttgattattaagagtgcaactgttggctttttatgcctttgaaaaagtgcaatcatgtagaatgatgatcactagatggtgaatgactgactgaacagtgatattacgaatcccctatgtgcacaaaatagagaggtcaggtgtagacctatgacaaggaaccacagacatttagttatcaatgcattagttctgatggaactgacattattttcaaaaagaaataatttttaaaagggtcgatttctaactgtgtgagtatataaacacacactctatttcttcataactaacctgccttgatgctagcactaaatcatgacaggcacctggttgaaagtggttgcaagaagccatcaattttaagatgcattgtgatttccaaatagtaaaatatagccaggcgcagtgtctcacacctgtaatcccaacactttgggaggctgaggcaggtgcaggagttcaagatcagcctggaccaacatggcaaaaccccatctctactaaaaatacaagaattagccagtatggtggtgcacacctgtgtatccagctacttgggaggctgaggcacgagaatcacttgaacccgagaggtgcaggttgcagtgagccgaaatcacaccactgcactccagccttggtgacagaaagagagatcctgtcccaaaaaaaaaaaaaagtaaaatacataccatatgatcacacatttccaaagatcattgatcaaggctgaccaatcctattaggtatataatggatctttataacagacaactccagtagttaccataagtgatcaaacttggcactggtgatactgggggaaatggatactatctgcttctgaggtattgcaagatgaagtacacatcaccatctatgaagtgttctggtaaaaaatgtttaagcctctatttccaacttcatgttacgagaaatgtgaaggagaggcccatatcaaatttcaccatgaggaatgaaactaatgtgtgacattctataaaacagctttcctaaactcttcaaaagtctggattttttcaagtctcatttttttagctcagcttaagggataaactctgaattaaaatcccctcaaattctttatactgtactagatcttatccagaatgaactatctgaaattcaaatggatgagtggttatgggaagcttttctgaattcattcctcaaaacggttgtgcctctcctaagaattcaccagtagtaatactaataataaagacaatatgaacaatagctaatatgtattaagcataggctacataccagatactcttccaaggatatgatgcatactaaatccatctaatctctgtaacagcattattagttaccatcagcatttgaaacatcatgtccagaagagataagcattttgctcaccatcctacaggtagtatggaggtgaaatggtgatgacagtatggtatttgccatggataagggttttcctacatttgttacattaacagagttactctctaggatgaacttactgaagtttaacaaagactgaatagtgttggaaggcttctgcacatttaacatatctggtataaattatcttatgctgttacaggcattagaaaattttgattccctcatttgccaaatcttgctatagtatgaatattctgctattctaatcagagaggtgcaagtgaagaatttcttatttaaattgtcacttgtctcatgtcttgaaaagtgtgagtcttgtctcaaattatttctgggaaagaacaaactttgttttcaattctcaatcatttatggactgataattttgtaaaacagaatgttatggaaatgtcaaattgctataaaagttccaaatatttactcactttccacgtttatctcacaattgacagatgacaattttatgactgcaccagtctctggataataatttgggtagcatttgtctaaaggccttcctataattctaattcaaatgatttctcatttggatgaattctctgatgtactctaagatatttactgtgtctataagccttcccaaattccttatgtgcataggattacacagcagtatgaattctctgatgtgcagcaagaactgaattaagtttaggtccttcccacattcctcctatttaaactctttttaacaaataccaattatttgatgttaatcagaccttatgtcatgaatgaagatcttcacacattccttacatttaaatgattttacatcagtataaattgatatccaataagactgtacagaagtctaaaggccttttcatattaattatattcaaaatatttctcactagtatgaattgctggatagcaagataattgcccataaacagaaatgaatggcttttgcacaacccttacattcacaaggtttctcaagagtaagagttcttattatgataagttgtctatacacacacacaaaatattcttttacaactttcaatcataaggtttcatcagtatcaattttctcatttgagtaagttgtccacagaaaggcttccccacattcgttatatttgtagggtttatcattactatgagttctctcatgaacaagttttgagccacaagtaaaggtcttcccgaattccttacgttgataaagcttctcaccagtatgaaatctctgatgaacactaagttgatagccactaccaaaggccttcccacagtctttacattcataagacttctcattagtatggactctctcatgcttaactaggcttgaaccccaactgaaggccttcccacattccttacatttgaaaggtttctcaccggtatgaattttctgatgttgagtaaggtgatagccacgactaaaagccttcccacattctttacattcatagggtttctcccctgtatggattctttcatgttgaacaaggcttgatccacaattaaaagccttcccacattccttacattcatagggtttctcaccagtgtgaaatacctgatgtcgagtaagttgatacccactacaaaaggtctttccgcattctttacattcatgggatttctcaccagtatgaactctctcatgtttaacaaggcttgaaccccaactaaaggccttcccacattccttacattcaaaaggtttctcaccagtatggattttctgatgttgagaaaggtgatagccacgactaaaggcctttccacattctttacattcataaggtttctcaccagtatgaattctttcatgttgaataagacttgatccgcaattaaaagccttcccacattccttgcattcatagggtttctcaccagtatgaaatatctgatgtcgagtaagttgatagccccaacaaaaagcctttccacatattttacattcataaggtttcttaccagtatggattttctgatgctgagtaagctgatagccacgactgaaggccttcccacattctttacatttataaggtttctcacctgtatgaattatctcatgtttagcaaggcttgagccccaaaaaaaggccttcccacattccttacatttataagatttcacaccagtatgaattttctgatgttgggtaaggtgatagccacgactaaaggccttcccacattctttacattcatagggtttctcaccagtgtgaattctctcatgtttaacaaggcttgatccccagctaaaggtcttcccacattccttacactcatagggtttctcaccagtatgaaatctctgatgcacattgagttgataggcacttaaataattcttcccacattctttacattcaaagtgtttttcagctgtatgagttctctcatgttgaacaagttttgagccatgactgcaagccttcccacattccttacaaacataggatttctctgtattatgaattctttgatgtggagtaagagatttactttttctgtaagaaggtattttttcatagctgattatcatttgactgaagtatccctcttgatgtccttttagtccctcgaatatgcttttgcacttccaattatttctgaagatggatgcctcaaggccaagggttttacttttgtccttcatctcccactgggaaaaatttatttcaaaaatatcattttctgaaaatatttttttggtctcatacgtttttgactccaaatatcagtcatggttctggaattgcaagaactaattaatgctccatgggattcctctattggtgaagcacagaatccagaaaagccagaacagctctcgaacatcctgtagctgttattcaatgtaatgagacacattcactgtcaagattctcctgaaccttgatttctaaacatgcaaaaatccttttctcctcttcaaactccttcttagaaatctggcaacctggcagcacatgcagagtccaagaaccttaaggacaccggaaaaggacccagagacctgtggttagtttggacccagaggctgatgggaaacaagagcctggaaatgctcgcaggctgggagaggagcttctggcaggcaagctcgccccgcccctaaaag

SEQ ID NO: 14328 - RNA, 5052 nt, Homo sapiens
  source 1..5052: mol_type = other RNA
gctgggattacaggcatgagccaccgcgcccggccgtctttttttttttttcacttctctttagtcttttgataagctggtgaggtgcttttgcttgttccttaggaggggatttagtagatgctactttataagcttctttaactgtaaaatcctccttcattgtcaagtactagtaagcactggtgattccttgagatataatttcagaaatgttgggataaggcaccatgtctacatttcttggttaacaggcaaatgtggcacccagagggagtggcataatagccagttaccaataatatatcctgttaaaactcccaaagtactctgctttgtgttacagttgattattaagagtgcaactgttggctttttatgcctttgaaaaagtgcaatcatgtagaatgatgatcactagatggtgaatgactgactgaacagtgatattacgaatcccctatgtgcacaaaatagagaggtcaggtgtagacctatgacaaggaaccacagacatttagttatcaatgcattagttctgatggaactgacattattttcaaaaagaaataatttttaaaagggtcgatttctaactgtgtgagtatataaacacacactctatttcttcataactaacctgccttgatgctagcactaaatcatgacaggcacctggttgaaagtggttgcaagaagccatcaattttaagatgcattgtgatttccaaatagtaaaatatagccaggcgcagtgtctcacacctgtaatcccaacactttgggaggctgaggcaggtgcaggagttcaagatcagcctggaccaacatggcaaaaccccatctctactaaaaatacaagaattagccagtatggtggtgcacacctgtgtatccagctacttgggaggctgaggcacgagaatcacttgaacccgagaggtgcaggttgcagtgagccgaaatcacaccactgcactccagccttggtgacagaaagagagatcctgtcccaaaaaaaaaaaaaagtaaaatacataccatatgatcacacatttccaaagatcattgatcaaggctgaccaatcctattaggtatataatggatctttataacagacaactccagtagttaccataagtgatcaaacttggcactggtgatactgggggaaatggatactatctgcttctgaggtattgcaagatgaagtacacatcaccatctatgaagtgttctggtaaaaaatgtttaagcctctatttccaacttcatgttacgagaaatgtgaaggagaggcccatatcaaatttcaccatgaggaatgaaactaatgtgtgacattctataaaacagctttcctaaactcttcaaaagtctggattttttcaagtctcatttttttagctcagcttaagggataaactctgaattaaaatcccctcaaattctttatactgtactagatcttatccagaatgaactatctgaaattcaaatggatgagtggttatgggaagcttttctgaattcattcctcaaaacggttgtgcctctcctaagaattcaccagtagtaatactaataataaagacaatatgaacaatagctaatatgtattaagcataggctacataccagatactcttccaaggatatgatgcatactaaatccatctaatctctgtaacagcattattagttaccatcagcatttgaaacatcatgtccagaagagataagcattttgctcaccatcctacaggtagtatggaggtgaaatggtgatgacagtatggtatttgccatggataagggttttcctacatttgttacattaacagagttactctctaggatgaacttactgaagtttaacaaagactgaatagtgttggaaggcttctgcacatttaacatatctggtataaattatcttatgctgttacaggcattagaaaattttgattccctcatttgccaaatcttgctatagtatgaatattctgctattctaatcagagaggtgcaagtgaagaatttcttatttaaattgtcacttgtctcatgtcttgaaaagtgtgagtcttgtctcaaattatttctgggaaagaacaaactttgttttcaattctcaatcatttatggactgataattttgtaaaacagaatgttatggaaatgtcaaattgctataaaagttccaaatatttactcactttccacgtttatctcacaattgacagatgacaattttatgactgcaccagtctctggataataatttgggtagcatttgtctaaaggccttcctataattctaattcaaatgatttctcatttggatgaattctctgatgtactctaagatatttactgtgtctataagccttcccaaattccttatgtgcataggattacacagcagtatgaattctctgatgtgcagcaagaactgaattaagtttaggtccttcccacattcctcctatttaaactctttttaacaaataccaattatttgatgttaatcagaccttatgtcatgaatgaagatcttcacacattccttacatttaaatgattttacatcagtataaattgatatccaataagactgtacagaagtctaaaggccttttcatattaattatattcaaaatatttctcactagtatgaattgctggatagcaagataattgcccataaacagaaatgaatggcttttgcacaacccttacattcacaaggtttctcaagagtaagagttcttattatgataagttgtctatacacacacacaaaatattcttttacaactttcaatcataaggtttcatcagtatcaattttctcatttgagtaagttgtccacagaaaggcttccccacattcgttatatttgtagggtttatcattactatgagttctctcatgaacaagttttgagccacaagtaaaggtcttcccgaattccttacgttgataaagcttctcaccagtatgaaatctctgatgaacactaagttgatagccactaccaaaggccttcccacagtctttacattcataagacttctcattagtatggactctctcatgcttaactaggcttgaaccccaactgaaggccttcccacattccttacatttgaaaggtttctcaccggtatgaattttctgatgttgagtaaggtgatagccacgactaaaagccttcccacattctttacattcatagggtttctcccctgtatggattctttcatgttgaacaaggcttgatccacaattaaaagccttcccacattccttacattcatagggtttctcaccagtgtgaaatacctgatgtcgagtaagttgatacccactacaaaaggtctttccgcattctttacattcatgggatttctcaccagtatgaactctctcatgtttaacaaggcttgaaccccaactaaaggccttcccacattccttacattcaaaaggtttctcaccagtatggattttctgatgttgagaaaggtgatagccacgactaaaggcctttccacattctttacattcataaggtttctcaccagtatgaattctttcatgttgaataagacttgatccgcaattaaaagccttcccacattccttgcattcatagggtttctcaccagtatgaaatatctgatgtcgagtaagttgatagccccaacaaaaagcctttccacatattttacattcataaggtttcttaccagtatggattttctgatgctgagtaagctgatagccacgactgaaggccttcccacattctttacatttataaggtttctcacctgtatgaattatctcatgtttagcaaggcttgagccccaaaaaaaggccttcccacattccttacatttataagatttcacaccagtatgaattttctgatgttgggtaaggtgatagccacgactaaaggccttcccacattctttacattcatagggtttctcaccagtgtgaattctctcatgtttaacaaggcttgatccccagctaaaggtcttcccacattccttacactcatagggtttctcaccagtatgaaatctctgatgcacattgagttgataggcacttaaataattcttcccacattctttacattcaaagtgtttttcagctgtatgagttctctcatgttgaacaagttttgagccatgactgcaagccttcccacattccttacaaacataggatttctctgtattatgaattctttgatgtggagtaagagatttactttttctgtaagaaggtattttttcatagctgattatcatttgactgaagtatccctcttgatgtccttttagtccctcgaatatgcttttgcacttccaattatttctgaagatggatgcctcaaggccaagggttttacttttgtccttcatctcccactgggaaaaatttatttcaaaaatatcattttctgaaaatatttttttggtctcatacgtttttgactccaaatatcagtcatggttctggaattgcaagaactaattaatgctccatgggattcctctattggtgaagcacagaatccagaaaagccagaacagctctcgaacatcctgtagctgttattcaatgtaatgagacacattcactgtcaagattctcctgaaccttgatttctaaacatgcaaaaatccttttctcctcttcaaactccttcttagaaatctggcaacctggcagcactctagaacttccccatcaggtcttgacaagatcctgtcccgcggacacttccagatctaaaattctcatccttcttgcttgaaacgttcattatggggcttagcatagacttctttcttgcggtcatttaattgtggcaggcccgaagacaggctaaagggaaccatgcagagtccaagaaccttaaggacaccggaaaaggacccagagacctgtggttagtttggacccagaggctgatgggaaacaagagcctggaaatgctcgcaggctgggagaggagcttct

SEQ ID NO: 14329 - RNA, 5244 nt, Homo sapiens
  source 1..5244: mol_type = other RNA
gctgggattacaggcatgagccaccgcgcccggccgtctttttttttttttcacttctctttagtcttttgataagctggtgaggtgcttttgcttgttccttaggaggggatttagtagatgctactttataagcttctttaactgtaaaatcctccttcattgtcaagtactagtaagcactggtgattccttgagatataatttcagaaatgttgggataaggcaccatgtctacatttcttggttaacaggcaaatgtggcacccagagggagtggcataatagccagttaccaataatatatcctgttaaaactcccaaagtactctgctttgtgttacagttgattattaagagtgcaactgttggctttttatgcctttgaaaaagtgcaatcatgtagaatgatgatcactagatggtgaatgactgactgaacagtgatattacgaatcccctatgtgcacaaaatagagaggtcaggtgtagacctatgacaaggaaccacagacatttagttatcaatgcattagttctgatggaactgacattattttcaaaaagaaataatttttaaaagggtcgatttctaactgtgtgagtatataaacacacactctatttcttcataactaacctgccttgatgctagcactaaatcatgacaggcacctggttgaaagtggttgcaagaagccatcaattttaagatgcattgtgatttccaaatagtaaaatatagccaggcgcagtgtctcacacctgtaatcccaacactttgggaggctgaggcaggtgcaggagttcaagatcagcctggaccaacatggcaaaaccccatctctactaaaaatacaagaattagccagtatggtggtgcacacctgtgtatccagctacttgggaggctgaggcacgagaatcacttgaacccgagaggtgcaggttgcagtgagccgaaatcacaccactgcactccagccttggtgacagaaagagagatcctgtcccaaaaaaaaaaaaaagtaaaatacataccatatgatcacacatttccaaagatcattgatcaaggctgaccaatcctattaggtatataatggatctttataacagacaactccagtagttaccataagtgatcaaacttggcactggtgatactgggggaaatggatactatctgcttctgaggtattgcaagatgaagtacacatcaccatctatgaagtgttctggtaaaaaatgtttaagcctctatttccaacttcatgttacgagaaatgtgaaggagaggcccatatcaaatttcaccatgaggaatgaaactaatgtgtgacattctataaaacagctttcctaaactcttcaaaagtctggattttttcaagtctcatttttttagctcagcttaagggataaactctgaattaaaatcccctcaaattctttatactgtactagatcttatccagaatgaactatctgaaattcaaatggatgagtggttatgggaagcttttctgaattcattcctcaaaacggttgtgcctctcctaagaattcaccagtagtaatactaataataaagacaatatgaacaatagctaatatgtattaagcataggctacataccagatactcttccaaggatatgatgcatactaaatccatctaatctctgtaacagcattattagttaccatcagcatttgaaacatcatgtccagaagagataagcattttgctcaccatcctacaggtagtatggaggtgaaatggtgatgacagtatggtatttgccatggataagggttttcctacatttgttacattaacagagttactctctaggatgaacttactgaagtttaacaaagactgaatagtgttggaaggcttctgcacatttaacatatctggtataaattatcttatgctgttacaggcattagaaaattttgattccctcatttgccaaatcttgctatagtatgaatattctgctattctaatcagagaggtgcaagtgaagaatttcttatttaaattgtcacttgtctcatgtcttgaaaagtgtgagtcttgtctcaaattatttctgggaaagaacaaactttgttttcaattctcaatcatttatggactgataattttgtaaaacagaatgttatggaaatgtcaaattgctataaaagttccaaatatttactcactttccacgtttatctcacaattgacagatgacaattttatgactgcaccagtctctggataataatttgggtagcatttgtctaaaggccttcctataattctaattcaaatgatttctcatttggatgaattctctgatgtactctaagatatttactgtgtctataagccttcccaaattccttatgtgcataggattacacagcagtatgaattctctgatgtgcagcaagaactgaattaagtttaggtccttcccacattcctcctatttaaactctttttaacaaataccaattatttgatgttaatcagaccttatgtcatgaatgaagatcttcacacattccttacatttaaatgattttacatcagtataaattgatatccaataagactgtacagaagtctaaaggccttttcatattaattatattcaaaatatttctcactagtatgaattgctggatagcaagataattgcccataaacagaaatgaatggcttttgcacaacccttacattcacaaggtttctcaagagtaagagttcttattatgataagttgtctatacacacacacaaaatattcttttacaactttcaatcataaggtttcatcagtatcaattttctcatttgagtaagttgtccacagaaaggcttccccacattcgttatatttgtagggtttatcattactatgagttctctcatgaacaagttttgagccacaagtaaaggtcttcccgaattccttacgttgataaagcttctcaccagtatgaaatctctgatgaacactaagttgatagccactaccaaaggccttcccacagtctttacattcataagacttctcattagtatggactctctcatgcttaactaggcttgaaccccaactgaaggccttcccacattccttacatttgaaaggtttctcaccggtatgaattttctgatgttgagtaaggtgatagccacgactaaaagccttcccacattctttacattcatagggtttctcccctgtatggattctttcatgttgaacaaggcttgatccacaattaaaagccttcccacattccttacattcatagggtttctcaccagtgtgaaatacctgatgtcgagtaagttgatacccactacaaaaggtctttccgcattctttacattcatgggatttctcaccagtatgaactctctcatgtttaacaaggcttgaaccccaactaaaggccttcccacattccttacattcaaaaggtttctcaccagtatggattttctgatgttgagaaaggtgatagccacgactaaaggcctttccacattctttacattcataaggtttctcaccagtatgaattctttcatgttgaataagacttgatccgcaattaaaagccttcccacattccttgcattcatagggtttctcaccagtatgaaatatctgatgtcgagtaagttgatagccccaacaaaaagcctttccacatattttacattcataaggtttcttaccagtatggattttctgatgctgagtaagctgatagccacgactgaaggccttcccacattctttacatttataaggtttctcacctgtatgaattatctcatgtttagcaaggcttgagccccaaaaaaaggccttcccacattccttacatttataagatttcacaccagtatgaattttctgatgttgggtaaggtgatagccacgactaaaggccttcccacattctttacattcatagggtttctcaccagtgtgaattctctcatgtttaacaaggcttgatccccagctaaaggtcttcccacattccttacactcatagggtttctcaccagtatgaaatctctgatgcacattgagttgataggcacttaaataattcttcccacattctttacattcaaagtgtttttcagctgtatgagttctctcatgttgaacaagttttgagccatgactgcaagccttcccacattccttacaaacataggatttctctgtattatgaattctttgatgtggagtaagagatttactttttctgtaagaaggtattttttcatagctgattatcatttgactgaagtatccctcttgatgtccttttagtccctcgaatatgcttttgcacttccaattatttctgaagatggatgcctcaaggccaagggttttacttttgtccttcatctcccactgggaaaaatttatttcaaaaatatcattttctgaaaatatttttttggtctcatacgtttttgactccaaatatcagtcatggttctggaattgcaagaactaattaatgctccatgggattcctctattggtgaagcacagaatccagaaaagccagaactgtagtcccagctactcaggaggctgaggcaggagaatagcgtgaacccaggaggcggagcttgcagtgagccaagatcgcaccactgcactccagcctgggcgacagagcgagactccatcagctctcgaacatcctgtagctgttattcaatgtaatgagacacattcactgtcaagattctcctgaaccttgatttctaaacatgcaaaaatccttttctcctcttcaaactccttcttagaaatctggcaacctggcagcacaccaaagagctcctagaggcccctcttctaggaatcccacctctagaacttccccatcaggtcttgacaagatcctgtcccgcggacacttccagatctaaaattctcatccttcttgcttgaaacgttcattatggggcttagcatagacttctttcttgcggtcatttaattgtggcaggcccgaagacaggctaaagggaaccatgcagagtccaagaaccttaaggacaccggaaaaggacccagagacctgtggttagtttggacccagaggctgatgggaaacaagagcctggaaatgctcgcaggctgggagaggagcttctggcaggcaagctcgccccgcccctaaaag

SEQ ID NO: 14330 - RNA, 5249 nt, Homo sapiens
  source 1..5249: mol_type = other RNA
gctgggattacaggcatgagccaccgcgcccggccgtctttttttttttttcacttctctttagtcttttgataagctggtgaggtgcttttgcttgttccttaggaggggatttagtagatgctactttataagcttctttaactgtaaaatcctccttcattgtcaagtactagtaagcactggtgattccttgagatataatttcagaaatgttgggataaggcaccatgtctacatttcttggttaacaggcaaatgtggcacccagagggagtggcataatagccagttaccaataatatatcctgttaaaactcccaaagtactctgctttgtgttacagttgattattaagagtgcaactgttggctttttatgcctttgaaaaagtgcaatcatgtagaatgatgatcactagatggtgaatgactgactgaacagtgatattacgaatcccctatgtgcacaaaatagagaggtcaggtgtagacctatgacaaggaaccacagacatttagttatcaatgcattagttctgatggaactgacattattttcaaaaagaaataatttttaaaagggtcgatttctaactgtgtgagtatataaacacacactctatttcttcataactaacctgccttgatgctagcactaaatcatgacaggcacctggttgaaagtggttgcaagaagccatcaattttaagatgcattgtgatttccaaatagtaaaatatagccaggcgcagtgtctcacacctgtaatcccaacactttgggaggctgaggcaggtgcaggagttcaagatcagcctggaccaacatggcaaaaccccatctctactaaaaatacaagaattagccagtatggtggtgcacacctgtgtatccagctacttgggaggctgaggcacgagaatcacttgaacccgagaggtgcaggttgcagtgagccgaaatcacaccactgcactccagccttggtgacagaaagagagatcctgtcccaaaaaaaaaaaaaagtaaaatacataccatatgatcacacatttccaaagatcattgatcaaggctgaccaatcctattaggtatataatggatctttataacagacaactccagtagttaccataagtgatcaaacttggcactggtgatactgggggaaatggatactatctgcttctgaggtattgcaagatgaagtacacatcaccatctatgaagtgttctggtaaaaaatgtttaagcctctatttccaacttcatgttacgagaaatgtgaaggagaggcccatatcaaatttcaccatgaggaatgaaactaatgtgtgacattctataaaacagctttcctaaactcttcaaaagtctggattttttcaagtctcatttttttagctcagcttaagggataaactctgaattaaaatcccctcaaattctttatactgtactagatcttatccagaatgaactatctgaaattcaaatggatgagtggttatgggaagcttttctgaattcattcctcaaaacggttgtgcctctcctaagaattcaccagtagtaatactaataataaagacaatatgaacaatagctaatatgtattaagcataggctacataccagatactcttccaaggatatgatgcatactaaatccatctaatctctgtaacagcattattagttaccatcagcatttgaaacatcatgtccagaagagataagcattttgctcaccatcctacaggtagtatggaggtgaaatggtgatgacagtatggtatttgccatggataagggttttcctacatttgttacattaacagagttactctctaggatgaacttactgaagtttaacaaagactgaatagtgttggaaggcttctgcacatttaacatatctggtataaattatcttatgctgttacaggcattagaaaattttgattccctcatttgccaaatcttgctatagtatgaatattctgctattctaatcagagaggtgcaagtgaagaatttcttatttaaattgtcacttgtctcatgtcttgaaaagtgtgagtcttgtctcaaattatttctgggaaagaacaaactttgttttcaattctcaatcatttatggactgataattttgtaaaacagaatgttatggaaatgtcaaattgctataaaagttccaaatatttactcactttccacgtttatctcacaattgacagatgacaattttatgactgcaccagtctctggataataatttgggtagcatttgtctaaaggccttcctataattctaattcaaatgatttctcatttggatgaattctctgatgtactctaagatatttactgtgtctataagccttcccaaattccttatgtgcataggattacacagcagtatgaattctctgatgtgcagcaagaactgaattaagtttaggtccttcccacattcctcctatttaaactctttttaacaaataccaattatttgatgttaatcagaccttatgtcatgaatgaagatcttcacacattccttacatttaaatgattttacatcagtataaattgatatccaataagactgtacagaagtctaaaggccttttcatattaattatattcaaaatatttctcactagtatgaattgctggatagcaagataattgcccataaacagaaatgaatggcttttgcacaacccttacattcacaaggtttctcaagagtaagagttcttattatgataagttgtctatacacacacacaaaatattcttttacaactttcaatcataaggtttcatcagtatcaattttctcatttgagtaagttgtccacagaaaggcttccccacattcgttatatttgtagggtttatcattactatgagttctctcatgaacaagttttgagccacaagtaaaggtcttcccgaattccttacgttgataaagcttctcaccagtatgaaatctctgatgaacactaagttgatagccactaccaaaggccttcccacagtctttacattcataagacttctcattagtatggactctctcatgcttaactaggcttgaaccccaactgaaggccttcccacattccttacatttgaaaggtttctcaccggtatgaattttctgatgttgagtaaggtgatagccacgactaaaagccttcccacattctttacattcatagggtttctcccctgtatggattctttcatgttgaacaaggcttgatccacaattaaaagccttcccacattccttacattcatagggtttctcaccagtgtgaaatacctgatgtcgagtaagttgatacccactacaaaaggtctttccgcattctttacattcatgggatttctcaccagtatgaactctctcatgtttaacaaggcttgaaccccaactaaaggccttcccacattccttacattcaaaaggtttctcaccagtatggattttctgatgttgagaaaggtgatagccacgactaaaggcctttccacattctttacattcataaggtttctcaccagtatgaattctttcatgttgaataagacttgatccgcaattaaaagccttcccacattccttgcattcatagggtttctcaccagtatgaaatatctgatgtcgagtaagttgatagccccaacaaaaagcctttccacatattttacattcataaggtttcttaccagtatggattttctgatgctgagtaagctgatagccacgactgaaggccttcccacattctttacatttataaggtttctcacctgtatgaattatctcatgtttagcaaggcttgagccccaaaaaaaggccttcccacattccttacatttataagatttcacaccagtatgaattttctgatgttgggtaaggtgatagccacgactaaaggccttcccacattctttacattcatagggtttctcaccagtgtgaattctctcatgtttaacaaggcttgatccccagctaaaggtcttcccacattccttacactcatagggtttctcaccagtatgaaatctctgatgcacattgagttgataggcacttaaataattcttcccacattctttacattcaaagtgtttttcagctgtatgagttctctcatgttgaacaagttttgagccatgactgcaagccttcccacattccttacaaacataggatttctctgtattatgaattctttgatgtggagtaagagatttactttttctgtaagaaggtattttttcatagctgattatcatttgactgaagtatccctcttgatgtccttttagtccctcgaatatgcttttgcacttccaattatttctgaagatggatgcctcaaggccaagggttttacttttgtccttcatctcccactgggaaaaatttatttcaaaaatatcattttctgaaaatatttttttggtctcatacgtttttgactccaaatccagtgacaccaagttactatagttctccaacattacatccacgtacaagtccctctgagcagggtccaggcattcccactcctcctgagagaagtcgatggccacatccctgaatgtcaccaacccatcagtcatggttctggaattgcaagaactaattaatgctccatgggattcctctattggtgaagcacagaatccagaaaagccagaacagctctcgaacatcctgtagctgttattcaatgtaatgagacacattcactgtcaagattctcctgaaccttgatttctaaacatgcaaaaatccttttctcctcttcaaactccttcttagaaatctggcaacctggcagcacaccaaagagctcctagaggcccctcttctaggaatcccacctctagaacttccccatcaggtcttgacaagatcctgtcccgcggacacttccagatctaaaattctcatccttcttgcttgaaacgttcattatggggcttagcatagacttctttcttgcggtcatttaattgtggcaggcccgaagacaggctaaagggaaccatgcagagtccaagaaccttaaggacaccggaaaaggacccagagacctgtggttagtttggacccagaggctgatgggaaacaagagcctggaaatgctcgcaggctgggagaggagcttctggcaggcaagctcgccccgcccctaaaag

SEQ ID NO: 14331 - RNA, 5043 nt, Homo sapiens
  source 1..5043: mol_type = other RNA
gctgggattacaggcatgagccaccgcgcccggccgtctttttttttttttcacttctctttagtcttttgataagctggtgaggtgcttttgcttgttccttaggaggggatttagtagatgctactttataagcttctttaactgtaaaatcctccttcattgtcaagtactagtaagcactggtgattccttgagatataatttcagaaatgttgggataaggcaccatgtctacatttcttggttaacaggcaaatgtggcacccagagggagtggcataatagccagttaccaataatatatcctgttaaaactcccaaagtactctgctttgtgttacagttgattattaagagtgcaactgttggctttttatgcctttgaaaaagtgcaatcatgtagaatgatgatcactagatggtgaatgactgactgaacagtgatattacgaatcccctatgtgcacaaaatagagaggtcaggtgtagacctatgacaaggaaccacagacatttagttatcaatgcattagttctgatggaactgacattattttcaaaaagaaataatttttaaaagggtcgatttctaactgtgtgagtatataaacacacactctatttcttcataactaacctgccttgatgctagcactaaatcatgacaggcacctggttgaaagtggttgcaagaagccatcaattttaagatgcattgtgatttccaaatagtaaaatatagccaggcgcagtgtctcacacctgtaatcccaacactttgggaggctgaggcaggtgcaggagttcaagatcagcctggaccaacatggcaaaaccccatctctactaaaaatacaagaattagccagtatggtggtgcacacctgtgtatccagctacttgggaggctgaggcacgagaatcacttgaacccgagaggtgcaggttgcagtgagccgaaatcacaccactgcactccagccttggtgacagaaagagagatcctgtcccaaaaaaaaaaaaaagtaaaatacataccatatgatcacacatttccaaagatcattgatcaaggctgaccaatcctattaggtatataatggatctttataacagacaactccagtagttaccataagtgatcaaacttggcactggtgatactgggggaaatggatactatctgcttctgaggtattgcaagatgaagtacacatcaccatctatgaagtgttctggtaaaaaatgtttaagcctctatttccaacttcatgttacgagaaatgtgaaggagaggcccatatcaaatttcaccatgaggaatgaaactaatgtgtgacattctataaaacagctttcctaaactcttcaaaagtctggattttttcaagtctcatttttttagctcagcttaagggataaactctgaattaaaatcccctcaaattctttatactgtactagatcttatccagaatgaactatctgaaattcaaatggatgagtggttatgggaagcttttctgaattcattcctcaaaacggttgtgcctctcctaagaattcaccagtagtaatactaataataaagacaatatgaacaatagctaatatgtattaagcataggctacataccagatactcttccaaggatatgatgcatactaaatccatctaatctctgtaacagcattattagttaccatcagcatttgaaacatcatgtccagaagagataagcattttgctcaccatcctacaggtagtatggaggtgaaatggtgatgacagtatggtatttgccatggataagggttttcctacatttgttacattaacagagttactctctaggatgaacttactgaagtttaacaaagactgaatagtgttggaaggcttctgcacatttaacatatctggtataaattatcttatgctgttacaggcattagaaaattttgattccctcatttgccaaatcttgctatagtatgaatattctgctattctaatcagagaggtgcaagtgaagaatttcttatttaaattgtcacttgtctcatgtcttgaaaagtgtgagtcttgtctcaaattatttctgggaaagaacaaactttgttttcaattctcaatcatttatggactgataattttgtaaaacagaatgttatggaaatgtcaaattgctataaaagttccaaatatttactcactttccacgtttatctcacaattgacagatgacaattttatgactgcaccagtctctggataataatttgggtagcatttgtctaaaggccttcctataattctaattcaaatgatttctcatttggatgaattctctgatgtactctaagatatttactgtgtctataagccttcccaaattccttatgtgcataggattacacagcagtatgaattctctgatgtgcagcaagaactgaattaagtttaggtccttcccacattcctcctatttaaactctttttaacaaataccaattatttgatgttaatcagaccttatgtcatgaatgaagatcttcacacattccttacatttaaatgattttacatcagtataaattgatatccaataagactgtacagaagtctaaaggccttttcatattaattatattcaaaatatttctcactagtatgaattgctggatagcaagataattgcccataaacagaaatgaatggcttttgcacaacccttacattcacaaggtttctcaagagtaagagttcttattatgataagttgtctatacacacacacaaaatattcttttacaactttcaatcataaggtttcatcagtatcaattttctcatttgagtaagttgtccacagaaaggcttccccacattcgttatatttgtagggtttatcattactatgagttctctcatgaacaagttttgagccacaagtaaaggtcttcccgaattccttacgttgataaagcttctcaccagtatgaaatctctgatgaacactaagttgatagccactaccaaaggccttcccacagtctttacattcataagacttctcattagtatggactctctcatgcttaactaggcttgaaccccaactgaaggccttcccacattccttacatttgaaaggtttctcaccggtatgaattttctgatgttgagtaaggtgatagccacgactaaaagccttcccacattctttacattcatagggtttctcccctgtatggattctttcatgttgaacaaggcttgatccacaattaaaagccttcccacattccttacattcatagggtttctcaccagtgtgaaatacctgatgtcgagtaagttgatacccactacaaaaggtctttccgcattctttacattcatgggatttctcaccagtatgaactctctcatgtttaacaaggcttgaaccccaactaaaggccttcccacattccttacattcaaaaggtttctcaccagtatggattttctgatgttgagaaaggtgatagccacgactaaaggcctttccacattctttacattcataaggtttctcaccagtatgaattctttcatgttgaataagacttgatccgcaattaaaagccttcccacattccttgcattcatagggtttctcaccagtatgaaatatctgatgtcgagtaagttgatagccccaacaaaaagcctttccacatattttacattcataaggtttcttaccagtatggattttctgatgctgagtaagctgatagccacgactgaaggccttcccacattctttacatttataaggtttctcacctgtatgaattatctcatgtttagcaaggcttgagccccaaaaaaaggccttcccacattccttacatttataagatttcacaccagtatgaattttctgatgttgggtaaggtgatagccacgactaaaggccttcccacattctttacattcatagggtttctcaccagtgtgaattctctcatgtttaacaaggcttgatccccagctaaaggtcttcccacattccttacactcatagggtttctcaccagtatgaaatctctgatgcacattgagttgataggcacttaaataattcttcccacattctttacattcaaagtgtttttcagctgtatgagttctctcatgttgaacaagttttgagccatgactgcaagccttcccacattccttacaaacataggatttctctgtattatgaattctttgatgtggagtaagagatttactttttctgtaagaaggtattttttcatagctgattatcatttgactgaagtatccctcttgatgtccttttagtccctcgaatatgcttttgcacttccaattatttctgaagatggatgcctcaaggccaagggttttacttttgtccttcatctcccactgggaaaaatttatttcaaaaatatcattttctgaaaatatttttttggtctcatacgtttttgactccaaatccagtgacaccaagttactatagttctccaacattacatccacgtacaagtccctctgagcagggtccaggcattcccactcctcctgagagaagtcgatggccacatccctgaatgtcaccaacccatcagtcatggttctggaattgcaagaactaattaatgctccatgggattcctctattggtgaagcacagaatccagaaaagccagaacagctctcgaacatcctgtagctgttattcaatgtaatgagacacattcactgtcaagattctcctgaaccttgatttctaaacatgcaaaaatccttttctcctcttcaaactccttcttagaaatctggcaacctggcagcacatgcagagtccaagaaccttaaggacaccggaaaaggacccagagacctgtggttagtttggacccagaggctgatgggaaacaagagcctggaaatgctcgcaggctgggagaggagcttctggcaggcaagctcgccccgcccctaaaag

SEQ ID NO: 14332 - RNA, 5208 nt, Homo sapiens
  source 1..5208: mol_type = other RNA
gctgggattacaggcatgagccaccgcgcccggccgtctttttttttttttcacttctctttagtcttttgataagctggtgaggtgcttttgcttgttccttaggaggggatttagtagatgctactttataagcttctttaactgtaaaatcctccttcattgtcaagtactagtaagcactggtgattccttgagatataatttcagaaatgttgggataaggcaccatgtctacatttcttggttaacaggcaaatgtggcacccagagggagtggcataatagccagttaccaataatatatcctgttaaaactcccaaagtactctgctttgtgttacagttgattattaagagtgcaactgttggctttttatgcctttgaaaaagtgcaatcatgtagaatgatgatcactagatggtgaatgactgactgaacagtgatattacgaatcccctatgtgcacaaaatagagaggtcaggtgtagacctatgacaaggaaccacagacatttagttatcaatgcattagttctgatggaactgacattattttcaaaaagaaataatttttaaaagggtcgatttctaactgtgtgagtatataaacacacactctatttcttcataactaacctgccttgatgctagcactaaatcatgacaggcacctggttgaaagtggttgcaagaagccatcaattttaagatgcattgtgatttccaaatagtaaaatatagccaggcgcagtgtctcacacctgtaatcccaacactttgggaggctgaggcaggtgcaggagttcaagatcagcctggaccaacatggcaaaaccccatctctactaaaaatacaagaattagccagtatggtggtgcacacctgtgtatccagctacttgggaggctgaggcacgagaatcacttgaacccgagaggtgcaggttgcagtgagccgaaatcacaccactgcactccagccttggtgacagaaagagagatcctgtcccaaaaaaaaaaaaaagtaaaatacataccatatgatcacacatttccaaagatcattgatcaaggctgaccaatcctattaggtatataatggatctttataacagacaactccagtagttaccataagtgatcaaacttggcactggtgatactgggggaaatggatactatctgcttctgaggtattgcaagatgaagtacacatcaccatctatgaagtgttctggtaaaaaatgtttaagcctctatttccaacttcatgttacgagaaatgtgaaggagaggcccatatcaaatttcaccatgaggaatgaaactaatgtgtgacattctataaaacagctttcctaaactcttcaaaagtctggattttttcaagtctcatttttttagctcagcttaagggataaactctgaattaaaatcccctcaaattctttatactgtactagatcttatccagaatgaactatctgaaattcaaatggatgagtggttatgggaagcttttctgaattcattcctcaaaacggttgtgcctctcctaagaattcaccagtagtaatactaataataaagacaatatgaacaatagctaatatgtattaagcataggctacataccagatactcttccaaggatatgatgcatactaaatccatctaatctctgtaacagcattattagttaccatcagcatttgaaacatcatgtccagaagagataagcattttgctcaccatcctacaggtagtatggaggtgaaatggtgatgacagtatggtatttgccatggataagggttttcctacatttgttacattaacagagttactctctaggatgaacttactgaagtttaacaaagactgaatagtgttggaaggcttctgcacatttaacatatctggtataaattatcttatgctgttacaggcattagaaaattttgattccctcatttgccaaatcttgctatagtatgaatattctgctattctaatcagagaggtgcaagtgaagaatttcttatttaaattgtcacttgtctcatgtcttgaaaagtgtgagtcttgtctcaaattatttctgggaaagaacaaactttgttttcaattctcaatcatttatggactgataattttgtaaaacagaatgttatggaaatgtcaaattgctataaaagttccaaatatttactcactttccacgtttatctcacaattgacagatgacaattttatgactgcaccagtctctggataataatttgggtagcatttgtctaaaggccttcctataattctaattcaaatgatttctcatttggatgaattctctgatgtactctaagatatttactgtgtctataagccttcccaaattccttatgtgcataggattacacagcagtatgaattctctgatgtgcagcaagaactgaattaagtttaggtccttcccacattcctcctatttaaactctttttaacaaataccaattatttgatgttaatcagaccttatgtcatgaatgaagatcttcacacattccttacatttaaatgattttacatcagtataaattgatatccaataagactgtacagaagtctaaaggccttttcatattaattatattcaaaatatttctcactagtatgaattgctggatagcaagataattgcccataaacagaaatgaatggcttttgcacaacccttacattcacaaggtttctcaagagtaagagttcttattatgataagttgtctatacacacacacaaaatattcttttacaactttcaatcataaggtttcatcagtatcaattttctcatttgagtaagttgtccacagaaaggcttccccacattcgttatatttgtagggtttatcattactatgagttctctcatgaacaagttttgagccacaagtaaaggtcttcccgaattccttacgttgataaagcttctcaccagtatgaaatctctgatgaacactaagttgatagccactaccaaaggccttcccacagtctttacattcataagacttctcattagtatggactctctcatgcttaactaggcttgaaccccaactgaaggccttcccacattccttacatttgaaaggtttctcaccggtatgaattttctgatgttgagtaaggtgatagccacgactaaaagccttcccacattctttacattcatagggtttctcccctgtatggattctttcatgttgaacaaggcttgatccacaattaaaagccttcccacattccttacattcatagggtttctcaccagtgtgaaatacctgatgtcgagtaagttgatacccactacaaaaggtctttccgcattctttacattcatgggatttctcaccagtatgaactctctcatgtttaacaaggcttgaaccccaactaaaggccttcccacattccttacattcaaaaggtttctcaccagtatggattttctgatgttgagaaaggtgatagccacgactaaaggcctttccacattctttacattcataaggtttctcaccagtatgaattctttcatgttgaataagacttgatccgcaattaaaagccttcccacattccttgcattcatagggtttctcaccagtatgaaatatctgatgtcgagtaagttgatagccccaacaaaaagcctttccacatattttacattcataaggtttcttaccagtatggattttctgatgctgagtaagctgatagccacgactgaaggccttcccacattctttacatttataaggtttctcacctgtatgaattatctcatgtttagcaaggcttgagccccaaaaaaaggccttcccacattccttacatttataagatttcacaccagtatgaattttctgatgttgggtaaggtgatagccacgactaaaggccttcccacattctttacattcatagggtttctcaccagtgtgaattctctcatgtttaacaaggcttgatccccagctaaaggtcttcccacattccttacactcatagggtttctcaccagtatgaaatctctgatgcacattgagttgataggcacttaaataattcttcccacattctttacattcaaagtgtttttcagctgtatgagttctctcatgttgaacaagttttgagccatgactgcaagccttcccacattccttacaaacataggatttctctgtattatgaattctttgatgtggagtaagagatttactttttctgtaagaaggtattttttcatagctgattatcatttgactgaagtatccctcttgatgtccttttagtccctcgaatatgcttttgcacttccaattatttctgaagatggatgcctcaaggccaagggttttacttttgtccttcatctcccactgggaaaaatttatttcaaaaatatcattttctgaaaatatttttttggtctcatacgtttttgactccaaatccagtgacaccaagttactatagttctccaacattacatccacgtacaagtccctctgagcagggtccaggcattcccactcctcctgagagaagtcgatggccacatccctgaatgtcaccaacccatcagtcatggttctggaattgcaagaactaattaatgctccatgggattcctctattggtgaagcacagaatccagaaaagccagaacagctctcgaacatcctgtagctgttattcaatgtaatgagacacattcactgtcaagattctcctgaaccttgatttctaaacatgcaaaaatccttttctcctcttcaaactccttcttagaaatctggcaacctggcagcactctagaacttccccatcaggtcttgacaagatcctgtcccgcggacacttccagatctaaaattctcatccttcttgcttgaaacgttcattatggggcttagcatagacttctttcttgcggtcatttaattgtggcaggcccgaagacaggctaaagggaaccatgcagagtccaagaaccttaaggacaccggaaaaggacccagagacctgtggttagtttggacccagaggctgatgggaaacaagagcctggaaatgctcgcaggctgggagaggagcttctggcaggcaagctcgccccgcccctaaaag

SEQ ID NO: 14333 - RNA, 4979 nt, Homo sapiens
  source 1..4979: mol_type = other RNA
gctgggattacaggcatgagccaccgcgcccggccgtctttttttttttttcacttctctttagtcttttgataagctggtgaggtgcttttgcttgttccttaggaggggatttagtagatgctactttataagcttctttaactgtaaaatcctccttcattgtcaagtactagtaagcactggtgattccttgagatataatttcagaaatgttgggataaggcaccatgtctacatttcttggttaacaggcaaatgtggcacccagagggagtggcataatagccagttaccaataatatatcctgttaaaactcccaaagtactctgctttgtgttacagttgattattaagagtgcaactgttggctttttatgcctttgaaaaagtgcaatcatgtagaatgatgatcactagatggtgaatgactgactgaacagtgatattacgaatcccctatgtgcacaaaatagagaggtcaggtgtagacctatgacaaggaaccacagacatttagttatcaatgcattagttctgatggaactgacattattttcaaaaagaaataatttttaaaagggtcgatttctaactgtgtgagtatataaacacacactctatttcttcataactaacctgccttgatgctagcactaaatcatgacaggcacctggttgaaagtggttgcaagaagccatcaattttaagatgcattgtgatttccaaatagtaaaatatagccaggcgcagtgtctcacacctgtaatcccaacactttgggaggctgaggcaggtgcaggagttcaagatcagcctggaccaacatggcaaaaccccatctctactaaaaatacaagaattagccagtatggtggtgcacacctgtgtatccagctacttgggaggctgaggcacgagaatcacttgaacccgagaggtgcaggttgcagtgagccgaaatcacaccactgcactccagccttggtgacagaaagagagatcctgtcccaaaaaaaaaaaaaagtaaaatacataccatatgatcacacatttccaaagatcattgatcaaggctgaccaatcctattaggtatataatggatctttataacagacaactccagtagttaccataagtgatcaaacttggcactggtgatactgggggaaatggatactatctgcttctgaggtattgcaagatgaagtacacatcaccatctatgaagtgttctggtaaaaaatgtttaagcctctatttccaacttcatgttacgagaaatgtgaaggagaggcccatatcaaatttcaccatgaggaatgaaactaatgtgtgacattctataaaacagctttcctaaactcttcaaaagtctggattttttcaagtctcatttttttagctcagcttaagggataaactctgaattaaaatcccctcaaattctttatactgtactagatcttatccagaatgaactatctgaaattcaaatggatgagtggttatgggaagcttttctgaattcattcctcaaaacggttgtgcctctcctaagaattcaccagtagtaatactaataataaagacaatatgaacaatagctaatatgtattaagcataggctacataccagatactcttccaaggatatgatgcatactaaatccatctaatctctgtaacagcattattagttaccatcagcatttgaaacatcatgtccagaagagataagcattttgctcaccatcctacaggtagtatggaggtgaaatggtgatgacagtatggtatttgccatggataagggttttcctacatttgttacattaacagagttactctctaggatgaacttactgaagtttaacaaagactgaatagtgttggaaggcttctgcacatttaacatatctggtataaattatcttatgctgttacaggcattagaaaattttgattccctcatttgccaaatcttgctatagtatgaatattctgctattctaatcagagaggtgcaagtgaagaatttcttatttaaattgtcacttgtctcatgtcttgaaaagtgtgagtcttgtctcaaattatttctgggaaagaacaaactttgttttcaattctcaatcatttatggactgataattttgtaaaacagaatgttatggaaatgtcaaattgctataaaagttccaaatatttactcactttccacgtttatctcacaattgacagatgacaattttatgactgcaccagtctctggataataatttgggtagcatttgtctaaaggccttcctataattctaattcaaatgatttctcatttggatgaattctctgatgtactctaagatatttactgtgtctataagccttcccaaattccttatgtgcataggattacacagcagtatgaattctctgatgtgcagcaagaactgaattaagtttaggtccttcccacattcctcctatttaaactctttttaacaaataccaattatttgatgttaatcagaccttatgtcatgaatgaagatcttcacacattccttacatttaaatgattttacatcagtataaattgatatccaataagactgtacagaagtctaaaggccttttcatattaattatattcaaaatatttctcactagtatgaattgctggatagcaagataattgcccataaacagaaatgaatggcttttgcacaacccttacattcacaaggtttctcaagagtaagagttcttattatgataagttgtctatacacacacacaaaatattcttttacaactttcaatcataaggtttcatcagtatcaattttctcatttgagtaagttgtccacagaaaggcttccccacattcgttatatttgtagggtttatcattactatgagttctctcatgaacaagttttgagccacaagtaaaggtcttcccgaattccttacgttgataaagcttctcaccagtatgaaatctctgatgaacactaagttgatagccactaccaaaggccttcccacagtctttacattcataagacttctcattagtatggactctctcatgcttaactaggcttgaaccccaactgaaggccttcccacattccttacatttgaaaggtttctcaccggtatgaattttctgatgttgagtaaggtgatagccacgactaaaagccttcccacattctttacattcatagggtttctcccctgtatggattctttcatgttgaacaaggcttgatccacaattaaaagccttcccacattccttacattcatagggtttctcaccagtgtgaaatacctgatgtcgagtaagttgatacccactacaaaaggtctttccgcattctttacattcatgggatttctcaccagtatgaactctctcatgtttaacaaggcttgaaccccaactaaaggccttcccacattccttacattcaaaaggtttctcaccagtatggattttctgatgttgagaaaggtgatagccacgactaaaggcctttccacattctttacattcataaggtttctcaccagtatgaattctttcatgttgaataagacttgatccgcaattaaaagccttcccacattccttgcattcatagggtttctcaccagtatgaaatatctgatgtcgagtaagttgatagccccaacaaaaagcctttccacatattttacattcataaggtttcttaccagtatggattttctgatgctgagtaagctgatagccacgactgaaggccttcccacattctttacatttataaggtttctcacctgtatgaattatctcatgtttagcaaggcttgagccccaaaaaaaggccttcccacattccttacatttataagatttcacaccagtatgaattttctgatgttgggtaaggtgatagccacgactaaaggccttcccacattctttacattcatagggtttctcaccagtgtgaattctctcatgtttaacaaggcttgatccccagctaaaggtcttcccacattccttacactcatagggtttctcaccagtatgaaatctctgatgcacattgagttgataggcacttaaataattcttcccacattctttacattcaaagtgtttttcagctgtatgagttctctcatgttgaacaagttttgagccatgactgcaagccttcccacattccttacaaacataggatttctctgtattatgaattctttgatgtggagtaagagatttactttttctgtaagaaggtattttttcatagctgattatcatttgactgaagtatccctcttgatgtccttttagtccctcgaatatgcttttgcacttccaattatttctgaagatggatgcctcaaggccaagggttttacttttgtccttcatctcccactgggaaaaatttatttcaaaaatatcattttctgaaaatatttttttggtctcatacgtttttgactccaaatccagtgacaccaagttactatagttctccaacattacatccacgtacaagtccctctgagcagggtccaggcattcccactcctcctgagagaagtcgatggccacatccctgaatgtcaccaacccatcagtcatggttctggaattgcaagaactaattaatgctccatgggattcctctattggtgaagcacagaatccagaaaagccagaacagctctcgaacatcctgtagctgttattcaatgtaatgagacacattcactgtcaagattctcctggaagctcgtcaatggaacaagaagacctcaggttaagacttcctgtcgtaaggctgggcacagtggctcacgcctgtaatcctagcacttgaggagcccgaggcaggcagatcacttgagtccaggagttagagaccaggctgggcaacatagcaaaaccccctct

SEQ ID NO: 14334 - RNA, 5079 nt, Homo sapiens
  source 1..5079: mol_type = other RNA
gctgggattacaggcatgagccaccgcgcccggccgtctttttttttttttcacttctctttagtcttttgataagctggtgaggtgcttttgcttgttccttaggaggggatttagtagatgctactttataagcttctttaactgtaaaatcctccttcattgtcaagtactagtaagcactggtgattccttgagatataatttcagaaatgttgggataaggcaccatgtctacatttcttggttaacaggcaaatgtggcacccagagggagtggcataatagccagttaccaataatatatcctgttaaaactcccaaagtactctgctttgtgttacagttgattattaagagtgcaactgttggctttttatgcctttgaaaaagtgcaatcatgtagaatgatgatcactagatggtgaatgactgactgaacagtgatattacgaatcccctatgtgcacaaaatagagaggtcaggtgtagacctatgacaaggaaccacagacatttagttatcaatgcattagttctgatggaactgacattattttcaaaaagaaataatttttaaaagggtcgatttctaactgtgtgagtatataaacacacactctatttcttcataactaacctgccttgatgctagcactaaatcatgacaggcacctggttgaaagtggttgcaagaagccatcaattttaagatgcattgtgatttccaaatagtaaaatatagccaggcgcagtgtctcacacctgtaatcccaacactttgggaggctgaggcaggtgcaggagttcaagatcagcctggaccaacatggcaaaaccccatctctactaaaaatacaagaattagccagtatggtggtgcacacctgtgtatccagctacttgggaggctgaggcacgagaatcacttgaacccgagaggtgcaggttgcagtgagccgaaatcacaccactgcactccagccttggtgacagaaagagagatcctgtcccaaaaaaaaaaaaaagtaaaatacataccatatgatcacacatttccaaagatcattgatcaaggctgaccaatcctattaggtatataatggatctttataacagacaactccagtagttaccataagtgatcaaacttggcactggtgatactgggggaaatggatactatctgcttctgaggtattgcaagatgaagtacacatcaccatctatgaagtgttctggtaaaaaatgtttaagcctctatttccaacttcatgttacgagaaatgtgaaggagaggcccatatcaaatttcaccatgaggaatgaaactaatgtgtgacattctataaaacagctttcctaaactcttcaaaagtctggattttttcaagtctcatttttttagctcagcttaagggataaactctgaattaaaatcccctcaaattctttatactgtactagatcttatccagaatgaactatctgaaattcaaatggatgagtggttatgggaagcttttctgaattcattcctcaaaacggttgtgcctctcctaagaattcaccagtagtaatactaataataaagacaatatgaacaatagctaatatgtattaagcataggctacataccagatactcttccaaggatatgatgcatactaaatccatctaatctctgtaacagcattattagttaccatcagcatttgaaacatcatgtccagaagagataagcattttgctcaccatcctacaggtagtatggaggtgaaatggtgatgacagtatggtatttgccatggataagggttttcctacatttgttacattaacagagttactctctaggatgaacttactgaagtttaacaaagactgaatagtgttggaaggcttctgcacatttaacatatctggtataaattatcttatgctgttacaggcattagaaaattttgattccctcatttgccaaatcttgctatagtatgaatattctgctattctaatcagagaggtgcaagtgaagaatttcttatttaaattgtcacttgtctcatgtcttgaaaagtgtgagtcttgtctcaaattatttctgggaaagaacaaactttgttttcaattctcaatcatttatggactgataattttgtaaaacagaatgttatggaaatgtcaaattgctataaaagttccaaatatttactcactttccacgtttatctcacaattgacagatgacaattttatgactgcaccagtctctggataataatttgggtagcatttgtctaaaggccttcctataattctaattcaaatgatttctcatttggatgaattctctgatgtactctaagatatttactgtgtctataagccttcccaaattccttatgtgcataggattacacagcagtatgaattctctgatgtgcagcaagaactgaattaagtttaggtccttcccacattcctcctatttaaactctttttaacaaataccaattatttgatgttaatcagaccttatgtcatgaatgaagatcttcacacattccttacatttaaatgattttacatcagtataaattgatatccaataagactgtacagaagtctaaaggccttttcatattaattatattcaaaatatttctcactagtatgaattgctggatagcaagataattgcccataaacagaaatgaatggcttttgcacaacccttacattcacaaggtttctcaagagtaagagttcttattatgataagttgtctatacacacacacaaaatattcttttacaactttcaatcataaggtttcatcagtatcaattttctcatttgagtaagttgtccacagaaaggcttccccacattcgttatatttgtagggtttatcattactatgagttctctcatgaacaagttttgagccacaagtaaaggtcttcccgaattccttacgttgataaagcttctcaccagtatgaaatctctgatgaacactaagttgatagccactaccaaaggccttcccacagtctttacattcataagacttctcattagtatggactctctcatgcttaactaggcttgaaccccaactgaaggccttcccacattccttacatttgaaaggtttctcaccggtatgaattttctgatgttgagtaaggtgatagccacgactaaaagccttcccacattctttacattcatagggtttctcccctgtatggattctttcatgttgaacaaggcttgatccacaattaaaagccttcccacattccttacattcatagggtttctcaccagtgtgaaatacctgatgtcgagtaagttgatacccactacaaaaggtctttccgcattctttacattcatgggatttctcaccagtatgaactctctcatgtttaacaaggcttgaaccccaactaaaggccttcccacattccttacattcaaaaggtttctcaccagtatggattttctgatgttgagaaaggtgatagccacgactaaaggcctttccacattctttacattcataaggtttctcaccagtatgaattctttcatgttgaataagacttgatccgcaattaaaagccttcccacattccttgcattcatagggtttctcaccagtatgaaatatctgatgtcgagtaagttgatagccccaacaaaaagcctttccacatattttacattcataaggtttcttaccagtatggattttctgatgctgagtaagctgatagccacgactgaaggccttcccacattctttacatttataaggtttctcacctgtatgaattatctcatgtttagcaaggcttgagccccaaaaaaaggccttcccacattccttacatttataagatttcacaccagtatgaattttctgatgttgggtaaggtgatagccacgactaaaggccttcccacattctttacattcatagggtttctcaccagtgtgaattctctcatgtttaacaaggcttgatccccagctaaaggtcttcccacattccttacactcatagggtttctcaccagtatgaaatctctgatgcacattgagttgataggcacttaaataattcttcccacattctttacattcaaagtgtttttcagctgtatgagttctctcatgttgaacaagttttgagccatgactgcaagccttcccacattccttacaaacataggatttctctgtattatgaattctttgatgtggagtaagagatttactttttctgtaagaaggtattttttcatagctgattatcatttgactgaagtatccctcttgatgtccttttagtccctcgaatatgcttttgcacttccaattatttctgaagatggatgcctcaaggccaagggttttacttttgtccttcatctcccactgggaaaaatttatttcaaaaatatcattttctgaaaatatttttttggtctcatacgtttttgactccaaatccagtgacaccaagttactatagttctccaacattacatccacgtacaagtccctctgagcagggtccaggcattcccactcctcctgagagaagtcgatggccacatccctgaatgtcaccaacccatcagtcatggttctggaattgcaagaactaattaatgctccatgggattcctctattggtgaagcacagaatccagaaaagccagaacagctctcgaacatcctgtagctgttattcaatgtaatgagacacattcactgtcaagattctcctgtagtcccaggtactcgggagcctgaggtgggaggatcgcttgagcctaggaggccaaggctacagtgagccatgatcatgccactgcactccagcctaggcaaaaggccaagaacctgaaccttgatttctaaacatgcaaaaatccttttctcctcttcaaactccttcttagaaatctggcaacctggcagcacatgcagagtccaagaaccttaaggacaccggaaaaggacccagagacctgtggttagtttggacccagag

SEQ ID NO: 14335 - RNA, 5326 nt, Homo sapiens
  source 1..5326: mol_type = other RNA
gctgggattacaggcatgagccaccgcgcccggccgtctttttttttttttcacttctctttagtcttttgataagctggtgaggtgcttttgcttgttccttaggaggggatttagtagatgctactttataagcttctttaactgtaaaatcctccttcattgtcaagtactagtaagcactggtgattccttgagatataatttcagaaatgttgggataaggcaccatgtctacatttcttggttaacaggcaaatgtggcacccagagggagtggcataatagccagttaccaataatatatcctgttaaaactcccaaagtactctgctttgtgttacagttgattattaagagtgcaactgttggctttttatgcctttgaaaaagtgcaatcatgtagaatgatgatcactagatggtgaatgactgactgaacagtgatattacgaatcccctatgtgcacaaaatagagaggtcaggtgtagacctatgacaaggaaccacagacatttagttatcaatgcattagttctgatggaactgacattattttcaaaaagaaataatttttaaaagggtcgatttctaactgtgtgagtatataaacacacactctatttcttcataactaacctgccttgatgctagcactaaatcatgacaggcacctggttgaaagtggttgcaagaagccatcaattttaagatgcattgtgatttccaaatagtaaaatatagccaggcgcagtgtctcacacctgtaatcccaacactttgggaggctgaggcaggtgcaggagttcaagatcagcctggaccaacatggcaaaaccccatctctactaaaaatacaagaattagccagtatggtggtgcacacctgtgtatccagctacttgggaggctgaggcacgagaatcacttgaacccgagaggtgcaggttgcagtgagccgaaatcacaccactgcactccagccttggtgacagaaagagagatcctgtcccaaaaaaaaaaaaaagtaaaatacataccatatgatcacacatttccaaagatcattgatcaaggctgaccaatcctattaggtatataatggatctttataacagacaactccagtagttaccataagtgatcaaacttggcactggtgatactgggggaaatggatactatctgcttctgaggtattgcaagatgaagtacacatcaccatctatgaagtgttctggtaaaaaatgtttaagcctctatttccaacttcatgttacgagaaatgtgaaggagaggcccatatcaaatttcaccatgaggaatgaaactaatgtgtgacattctataaaacagctttcctaaactcttcaaaagtctggattttttcaagtctcatttttttagctcagcttaagggataaactctgaattaaaatcccctcaaattctttatactgtactagatcttatccagaatgaactatctgaaattcaaatggatgagtggttatgggaagcttttctgaattcattcctcaaaacggttgtgcctctcctaagaattcaccagtagtaatactaataataaagacaatatgaacaatagctaatatgtattaagcataggctacataccagatactcttccaaggatatgatgcatactaaatccatctaatctctgtaacagcattattagttaccatcagcatttgaaacatcatgtccagaagagataagcattttgctcaccatcctacaggtagtatggaggtgaaatggtgatgacagtatggtatttgccatggataagggttttcctacatttgttacattaacagagttactctctaggatgaacttactgaagtttaacaaagactgaatagtgttggaaggcttctgcacatttaacatatctggtataaattatcttatgctgttacaggcattagaaaattttgattccctcatttgccaaatcttgctatagtatgaatattctgctattctaatcagagaggtgcaagtgaagaatttcttatttaaattgtcacttgtctcatgtcttgaaaagtgtgagtcttgtctcaaattatttctgggaaagaacaaactttgttttcaattctcaatcatttatggactgataattttgtaaaacagaatgttatggaaatgtcaaattgctataaaagttccaaatatttactcactttccacgtttatctcacaattgacagatgacaattttatgactgcaccagtctctggataataatttgggtagcatttgtctaaaggccttcctataattctaattcaaatgatttctcatttggatgaattctctgatgtactctaagatatttactgtgtctataagccttcccaaattccttatgtgcataggattacacagcagtatgaattctctgatgtgcagcaagaactgaattaagtttaggtccttcccacattcctcctatttaaactctttttaacaaataccaattatttgatgttaatcagaccttatgtcatgaatgaagatcttcacacattccttacatttaaatgattttacatcagtataaattgatatccaataagactgtacagaagtctaaaggccttttcatattaattatattcaaaatatttctcactagtatgaattgctggatagcaagataattgcccataaacagaaatgaatggcttttgcacaacccttacattcacaaggtttctcaagagtaagagttcttattatgataagttgtctatacacacacacaaaatattcttttacaactttcaatcataaggtttcatcagtatcaattttctcatttgagtaagttgtccacagaaaggcttccccacattcgttatatttgtagggtttatcattactatgagttctctcatgaacaagttttgagccacaagtaaaggtcttcccgaattccttacgttgataaagcttctcaccagtatgaaatctctgatgaacactaagttgatagccactaccaaaggccttcccacagtctttacattcataagacttctcattagtatggactctctcatgcttaactaggcttgaaccccaactgaaggccttcccacattccttacatttgaaaggtttctcaccggtatgaattttctgatgttgagtaaggtgatagccacgactaaaagccttcccacattctttacattcatagggtttctcccctgtatggattctttcatgttgaacaaggcttgatccacaattaaaagccttcccacattccttacattcatagggtttctcaccagtgtgaaatacctgatgtcgagtaagttgatacccactacaaaaggtctttccgcattctttacattcatgggatttctcaccagtatgaactctctcatgtttaacaaggcttgaaccccaactaaaggccttcccacattccttacattcaaaaggtttctcaccagtatggattttctgatgttgagaaaggtgatagccacgactaaaggcctttccacattctttacattcataaggtttctcaccagtatgaattctttcatgttgaataagacttgatccgcaattaaaagccttcccacattccttgcattcatagggtttctcaccagtatgaaatatctgatgtcgagtaagttgatagccccaacaaaaagcctttccacatattttacattcataaggtttcttaccagtatggattttctgatgctgagtaagctgatagccacgactgaaggccttcccacattctttacatttataaggtttctcacctgtatgaattatctcatgtttagcaaggcttgagccccaaaaaaaggccttcccacattccttacatttataagatttcacaccagtatgaattttctgatgttgggtaaggtgatagccacgactaaaggccttcccacattctttacattcatagggtttctcaccagtgtgaattctctcatgtttaacaaggcttgatccccagctaaaggtcttcccacattccttacactcatagggtttctcaccagtatgaaatctctgatgcacattgagttgataggcacttaaataattcttcccacattctttacattcaaagtgtttttcagctgtatgagttctctcatgttgaacaagttttgagccatgactgcaagccttcccacattccttacaaacataggatttctctgtattatgaattctttgatgtggagtaagagatttactttttctgtaagaaggtattttttcatagctgattatcatttgactgaagtatccctcttgatgtccttttagtccctcgaatatgcttttgcacttccaattatttctgaagatggatgcctcaaggccaagggttttacttttgtccttcatctcccactgggaaaaatttatttcaaaaatatcattttctgaaaatatttttttggtctcatacgtttttgactccaaatccagtgacaccaagttactatagttctccaacattacatccacgtacaagtccctctgagcagggtccaggcattcccactcctcctgagagaagtcgatggccacatccctgaatgtcaccaacccatcagtcatggttctggaattgcaagaactaattaatgctccatgggattcctctattggtgaagcacagaatccagaaaagccagaacagctctcgaacatcctgtagctgttattcaatgtaatgagacacattcactgtcaagattctcctgtagtcccaggtactcgggagcctgaggtgggaggatcgcttgagcctaggaggccaaggctacagtgagccatgatcatgccactgcactccagcctaggcaaaaggccaagaacctgaaccttgatttctaaacatgcaaaaatccttttctcctcttcaaactccttcttagaaatctggcaacctggcagcactctagaacttccccatcaggtcttgacaagatcctgtcccgcggacacttccagatctaaaattctcatccttcttgcttgaaacgttcattatggggcttagcatagacttctttcttgcggtcatttaattgtggcaggcccgaagacaggctaaagggaaccatgcagagtccaagaaccttaaggacaccggaaaaggacccagagacctgtggttagtttggacccagaggctgatgggaaacaagagcctggaaatgctcgcaggctgggagaggagcttctggcaggcaagctcgccccgcccctaaaag

SEQ ID NO: 14336 - RNA, 5144 nt, Homo sapiens
  source 1..5144: mol_type = other RNA
gctgggattacaggcatgagccaccgcgcccggccgtctttttttttttttcacttctctttagtcttttgataagctggtgaggtgcttttgcttgttccttaggaggggatttagtagatgctactttataagcttctttaactgtaaaatcctccttcattgtcaagtactagtaagcactggtgattccttgagatataatttcagaaatgttgggataaggcaccatgtctacatttcttggttaacaggcaaatgtggcacccagagggagtggcataatagccagttaccaataatatatcctgttaaaactcccaaagtactctgctttgtgttacagttgattattaagagtgcaactgttggctttttatgcctttgaaaaagtgcaatcatgtagaatgatgatcactagatggtgaatgactgactgaacagtgatattacgaatcccctatgtgcacaaaatagagaggtcaggtgtagacctatgacaaggaaccacagacatttagttatcaatgcattagttctgatggaactgacattattttcaaaaagaaataatttttaaaagggtcgatttctaactgtgtgagtatataaacacacactctatttcttcataactaacctgccttgatgctagcactaaatcatgacaggcacctggttgaaagtggttgcaagaagccatcaattttaagatgcattgtgatttccaaatagtaaaatatagccaggcgcagtgtctcacacctgtaatcccaacactttgggaggctgaggcaggtgcaggagttcaagatcagcctggaccaacatggcaaaaccccatctctactaaaaatacaagaattagccagtatggtggtgcacacctgtgtatccagctacttgggaggctgaggcacgagaatcacttgaacccgagaggtgcaggttgcagtgagccgaaatcacaccactgcactccagccttggtgacagaaagagagatcctgtcccaaaaaaaaaaaaaagtaaaatacataccatatgatcacacatttccaaagatcattgatcaaggctgaccaatcctattaggtatataatggatctttataacagacaactccagtagttaccataagtgatcaaacttggcactggtgatactgggggaaatggatactatctgcttctgaggtattgcaagatgaagtacacatcaccatctatgaagtgttctggtaaaaaatgtttaagcctctatttccaacttcatgttacgagaaatgtgaaggagaggcccatatcaaatttcaccatgaggaatgaaactaatgtgtgacattctataaaacagctttcctaaactcttcaaaagtctggattttttcaagtctcatttttttagctcagcttaagggataaactctgaattaaaatcccctcaaattctttatactgtactagatcttatccagaatgaactatctgaaattcaaatggatgagtggttatgggaagcttttctgaattcattcctcaaaacggttgtgcctctcctaagaattcaccagtagtaatactaataataaagacaatatgaacaatagctaatatgtattaagcataggctacataccagatactcttccaaggatatgatgcatactaaatccatctaatctctgtaacagcattattagttaccatcagcatttgaaacatcatgtccagaagagataagcattttgctcaccatcctacaggtagtatggaggtgaaatggtgatgacagtatggtatttgccatggataagggttttcctacatttgttacattaacagagttactctctaggatgaacttactgaagtttaacaaagactgaatagtgttggaaggcttctgcacatttaacatatctggtataaattatcttatgctgttacaggcattagaaaattttgattccctcatttgccaaatcttgctatagtatgaatattctgctattctaatcagagaggtgcaagtgaagaatttcttatttaaattgtcacttgtctcatgtcttgaaaagtgtgagtcttgtctcaaattatttctgggaaagaacaaactttgttttcaattctcaatcatttatggactgataattttgtaaaacagaatgttatggaaatgtcaaattgctataaaagttccaaatatttactcactttccacgtttatctcacaattgacagatgacaattttatgactgcaccagtctctggataataatttgggtagcatttgtctaaaggccttcctataattctaattcaaatgatttctcatttggatgaattctctgatgtactctaagatatttactgtgtctataagccttcccaaattccttatgtgcataggattacacagcagtatgaattctctgatgtgcagcaagaactgaattaagtttaggtccttcccacattcctcctatttaaactctttttaacaaataccaattatttgatgttaatcagaccttatgtcatgaatgaagatcttcacacattccttacatttaaatgattttacatcagtataaattgatatccaataagactgtacagaagtctaaaggccttttcatattaattatattcaaaatatttctcactagtatgaattgctggatagcaagataattgcccataaacagaaatgaatggcttttgcacaacccttacattcacaaggtttctcaagagtaagagttcttattatgataagttgtctatacacacacacaaaatattcttttacaactttcaatcataaggtttcatcagtatcaattttctcatttgagtaagttgtccacagaaaggcttccccacattcgttatatttgtagggtttatcattactatgagttctctcatgaacaagttttgagccacaagtaaaggtcttcccgaattccttacgttgataaagcttctcaccagtatgaaatctctgatgaacactaagttgatagccactaccaaaggccttcccacagtctttacattcataagacttctcattagtatggactctctcatgcttaactaggcttgaaccccaactgaaggccttcccacattccttacatttgaaaggtttctcaccggtatgaattttctgatgttgagtaaggtgatagccacgactaaaagccttcccacattctttacattcatagggtttctcccctgtatggattctttcatgttgaacaaggcttgatccacaattaaaagccttcccacattccttacattcatagggtttctcaccagtgtgaaatacctgatgtcgagtaagttgatacccactacaaaaggtctttccgcattctttacattcatgggatttctcaccagtatgaactctctcatgtttaacaaggcttgaaccccaactaaaggccttcccacattccttacattcaaaaggtttctcaccagtatggattttctgatgttgagaaaggtgatagccacgactaaaggcctttccacattctttacattcataaggtttctcaccagtatgaattctttcatgttgaataagacttgatccgcaattaaaagccttcccacattccttgcattcatagggtttctcaccagtatgaaatatctgatgtcgagtaagttgatagccccaacaaaaagcctttccacatattttacattcataaggtttcttaccagtatggattttctgatgctgagtaagctgatagccacgactgaaggccttcccacattctttacatttataaggtttctcacctgtatgaattatctcatgtttagcaaggcttgagccccaaaaaaaggccttcccacattccttacatttataagatttcacaccagtatgaattttctgatgttgggtaaggtgatagccacgactaaaggccttcccacattctttacattcatagggtttctcaccagtgtgaattctctcatgtttaacaaggcttgatccccagctaaaggtcttcccacattccttacactcatagggtttctcaccagtatgaaatctctgatgcacattgagttgataggcacttaaataattcttcccacattctttacattcaaagtgtttttcagctgtatgagttctctcatgttgaacaagttttgagccatgactgcaagccttcccacattccttacaaacataggatttctctgtattatgaattctttgatgtggagtaagagatttactttttctgtaagaaggtattttttcatagctgattatcatttgactgaagtatccctcttgatgtccttttagtccctcgaatatgcttttgcacttccaattatttctgaagatggatgcctcaaggccaagggttttacttttgtccttcatctcccactgggaaaaatttatttcaaaaatatcattttctgaaaatatttttttggtctcatacgtttttgactccaaatccagtgacaccaagttactatagttctccaacattacatccacgtacaagtccctctgagcagggtccaggcattcccactcctcctgagagaagtcgatggccacatccctgaatgtcaccaacccatcagtcatggttctggaattgcaagaactaattaatgctccatgggattcctctattggtgaagcacagaatccagaaaagccagaactgaaccttgatttctaaacatgcaaaaatccttttctcctcttcaaactccttcttagaaatctggcaacctggcagcactctagaacttccccatcaggtcttgacaagatcctgtcccgcggacacttccagatctaaaattctcatccttcttgcttgaaacgttcattatggggcttagcatagacttctttcttgcggtcatttaattgtggcaggcccgaagacaggctaaagggaaccatgcagagtccaagaaccttaaggacaccggaaaaggacccagagacctgtggttagtttggacccagaggctgatgggaaacaagagcctggaaatgctcgcaggctgggagaggagcttctggcaggcaagctcgccccgcccctaaaag

SEQ ID NO: 14337 - RNA, 5371 nt, Homo sapiens
  source 1..5371: mol_type = other RNA
gctgggattacaggcatgagccaccgcgcccggccgtctttttttttttttcacttctctttagtcttttgataagctggtgaggtgcttttgcttgttccttaggaggggatttagtagatgctactttataagcttctttaactgtaaaatcctccttcattgtcaagtactagtaagcactggtgattccttgagatataatttcagaaatgttgggataaggcaccatgtctacatttcttggttaacaggcaaatgtggcacccagagggagtggcataatagccagttaccaataatatatcctgttaaaactcccaaagtactctgctttgtgttacagttgattattaagagtgcaactgttggctttttatgcctttgaaaaagtgcaatcatgtagaatgatgatcactagatggtgaatgactgactgaacagtgatattacgaatcccctatgtgcacaaaatagagaggtcaggtgtagacctatgacaaggaaccacagacatttagttatcaatgcattagttctgatggaactgacattattttcaaaaagaaataatttttaaaagggtcgatttctaactgtgtgagtatataaacacacactctatttcttcataactaacctgccttgatgctagcactaaatcatgacaggcacctggttgaaagtggttgcaagaagccatcaattttaagatgcattgtgatttccaaatagtaaaatatagccaggcgcagtgtctcacacctgtaatcccaacactttgggaggctgaggcaggtgcaggagttcaagatcagcctggaccaacatggcaaaaccccatctctactaaaaatacaagaattagccagtatggtggtgcacacctgtgtatccagctacttgggaggctgaggcacgagaatcacttgaacccgagaggtgcaggttgcagtgagccgaaatcacaccactgcactccagccttggtgacagaaagagagatcctgtcccaaaaaaaaaaaaaagtaaaatacataccatatgatcacacatttccaaagatcattgatcaaggctgaccaatcctattaggtatataatggatctttataacagacaactccagtagttaccataagtgatcaaacttggcactggtgatactgggggaaatggatactatctgcttctgaggtattgcaagatgaagtacacatcaccatctatgaagtgttctggtaaaaaatgtttaagcctctatttccaacttcatgttacgagaaatgtgaaggagaggcccatatcaaatttcaccatgaggaatgaaactaatgtgtgacattctataaaacagctttcctaaactcttcaaaagtctggattttttcaagtctcatttttttagctcagcttaagggataaactctgaattaaaatcccctcaaattctttatactgtactagatcttatccagaatgaactatctgaaattcaaatggatgagtggttatgggaagcttttctgaattcattcctcaaaacggttgtgcctctcctaagaattcaccagtagtaatactaataataaagacaatatgaacaatagctaatatgtattaagcataggctacataccagatactcttccaaggatatgatgcatactaaatccatctaatctctgtaacagcattattagttaccatcagcatttgaaacatcatgtccagaagagataagcattttgctcaccatcctacaggtagtatggaggtgaaatggtgatgacagtatggtatttgccatggataagggttttcctacatttgttacattaacagagttactctctaggatgaacttactgaagtttaacaaagactgaatagtgttggaaggcttctgcacatttaacatatctggtataaattatcttatgctgttacaggcattagaaaattttgattccctcatttgccaaatcttgctatagtatgaatattctgctattctaatcagagaggtgcaagtgaagaatttcttatttaaattgtcacttgtctcatgtcttgaaaagtgtgagtcttgtctcaaattatttctgggaaagaacaaactttgttttcaattctcaatcatttatggactgataattttgtaaaacagaatgttatggaaatgtcaaattgctataaaagttccaaatatttactcactttccacgtttatctcacaattgacagatgacaattttatgactgcaccagtctctggataataatttgggtagcatttgtctaaaggccttcctataattctaattcaaatgatttctcatttggatgaattctctgatgtactctaagatatttactgtgtctataagccttcccaaattccttatgtgcataggattacacagcagtatgaattctctgatgtgcagcaagaactgaattaagtttaggtccttcccacattcctcctatttaaactctttttaacaaataccaattatttgatgttaatcagaccttatgtcatgaatgaagatcttcacacattccttacatttaaatgattttacatcagtataaattgatatccaataagactgtacagaagtctaaaggccttttcatattaattatattcaaaatatttctcactagtatgaattgctggatagcaagataattgcccataaacagaaatgaatggcttttgcacaacccttacattcacaaggtttctcaagagtaagagttcttattatgataagttgtctatacacacacacaaaatattcttttacaactttcaatcataaggtttcatcagtatcaattttctcatttgagtaagttgtccacagaaaggcttccccacattcgttatatttgtagggtttatcattactatgagttctctcatgaacaagttttgagccacaagtaaaggtcttcccgaattccttacgttgataaagcttctcaccagtatgaaatctctgatgaacactaagttgatagccactaccaaaggccttcccacagtctttacattcataagacttctcattagtatggactctctcatgcttaactaggcttgaaccccaactgaaggccttcccacattccttacatttgaaaggtttctcaccggtatgaattttctgatgttgagtaaggtgatagccacgactaaaagccttcccacattctttacattcatagggtttctcccctgtatggattctttcatgttgaacaaggcttgatccacaattaaaagccttcccacattccttacattcatagggtttctcaccagtgtgaaatacctgatgtcgagtaagttgatacccactacaaaaggtctttccgcattctttacattcatgggatttctcaccagtatgaactctctcatgtttaacaaggcttgaaccccaactaaaggccttcccacattccttacattcaaaaggtttctcaccagtatggattttctgatgttgagaaaggtgatagccacgactaaaggcctttccacattctttacattcataaggtttctcaccagtatgaattctttcatgttgaataagacttgatccgcaattaaaagccttcccacattccttgcattcatagggtttctcaccagtatgaaatatctgatgtcgagtaagttgatagccccaacaaaaagcctttccacatattttacattcataaggtttcttaccagtatggattttctgatgctgagtaagctgatagccacgactgaaggccttcccacattctttacatttataaggtttctcacctgtatgaattatctcatgtttagcaaggcttgagccccaaaaaaaggccttcccacattccttacatttataagatttcacaccagtatgaattttctgatgttgggtaaggtgatagccacgactaaaggccttcccacattctttacattcatagggtttctcaccagtgtgaattctctcatgtttaacaaggcttgatccccagctaaaggtcttcccacattccttacactcatagggtttctcaccagtatgaaatctctgatgcacattgagttgataggcacttaaataattcttcccacattctttacattcaaagtgtttttcagctgtatgagttctctcatgttgaacaagttttgagccatgactgcaagccttcccacattccttacaaacataggatttctctgtattatgaattctttgatgtggagtaagagatttactttttctgtaagaaggtattttttcatagctgattatcatttgactgaagtatccctcttgatgtccttttagtccctcgaatatgcttttgcacttccaattatttctgaagatggatgcctcaaggccaagggttttacttttgtccttcatctcccactgggaaaaatttatttcaaaaatatcattttctgaaaatatttttttggtctcatacgtttttgactccaaatccagtgacaccaagttactatagttctccaacattacatccacgtacaagtccctctgagcagggtccaggcattcccactcctcctgagagaagtcgatggccacatccctgaatgtcaccaacccatcagtcatggttctggaattgcaagaactaattaatgctccatgggattcctctattggtgaagcacagaatccagaaaagccagaactgtagtcccagctactcaggaggctgaggcaggagaatagcgtgaacccaggaggcggagcttgcagtgagccaagatcgcaccactgcactccagcctgggcgacagagcgagactccatcagctctcgaacatcctgtagctgttattcaatgtaatgagacacattcactgtcaagattctcctgaaccttgatttctaaacatgcaaaaatccttttctcctcttcaaactccttcttagaaatctggcaacctggcagcacaccaaagagctcctagaggcccctcttctaggaatcccacctctagaacttccccatcaggtcttgacaagatcctgtcccgcggacacttccagatctaaaattctcatccttcttgcttgaaacgttcattatggggcttagcatagacttctttcttgcggtcatttaattgtggcaggcccgaagacaggctaaagggaaccatgcagagtccaagaaccttaaggacaccggaaaaggacccagagacctgtggttagtttggacccagaggctgatgggaaacaagagcctggaaatgctcgcaggctgggagaggagcttctggcaggcaagctcgccccgcccctaaaag

SEQ ID NO: 14338 - RNA, 5136 nt, Homo sapiens
  source 1..5136: mol_type = other RNA
gctgggattacaggcatgagccaccgcgcccggccgtctttttttttttttcacttctctttagtcttttgataagctggtgaggtgcttttgcttgttccttaggaggggatttagtagatgctactttataagcttctttaactgtaaaatcctccttcattgtcaagtactagtaagcactggtgattccttgagatataatttcagaaatgttgggataaggcaccatgtctacatttcttggttaacaggcaaatgtggcacccagagggagtggcataatagccagttaccaataatatatcctgttaaaactcccaaagtactctgctttgtgttacagttgattattaagagtgcaactgttggctttttatgcctttgaaaaagtgcaatcatgtagaatgatgatcactagatggtgaatgactgactgaacagtgatattacgaatcccctatgtgcacaaaatagagaggtcaggtgtagacctatgacaaggaaccacagacatttagttatcaatgcattagttctgatggaactgacattattttcaaaaagaaataatttttaaaagggtcgatttctaactgtgtgagtatataaacacacactctatttcttcataactaacctgccttgatgctagcactaaatcatgacaggcacctggttgaaagtggttgcaagaagccatcaattttaagatgcattgtgatttccaaatagtaaaatatagccaggcgcagtgtctcacacctgtaatcccaacactttgggaggctgaggcaggtgcaggagttcaagatcagcctggaccaacatggcaaaaccccatctctactaaaaatacaagaattagccagtatggtggtgcacacctgtgtatccagctacttgggaggctgaggcacgagaatcacttgaacccgagaggtgcaggttgcagtgagccgaaatcacaccactgcactccagccttggtgacagaaagagagatcctgtcccaaaaaaaaaaaaaagtaaaatacataccatatgatcacacatttccaaagatcattgatcaaggctgaccaatcctattaggtatataatggatctttataacagacaactccagtagttaccataagtgatcaaacttggcactggtgatactgggggaaatggatactatctgcttctgaggtattgcaagatgaagtacacatcaccatctatgaagtgttctggtaaaaaatgtttaagcctctatttccaacttcatgttacgagaaatgtgaaggagaggcccatatcaaatttcaccatgaggaatgaaactaatgtgtgacattctataaaacagctttcctaaactcttcaaaagtctggattttttcaagtctcatttttttagctcagcttaagggataaactctgaattaaaatcccctcaaattctttatactgtactagatcttatccagaatgaactatctgaaattcaaatggatgagtggttatgggaagcttttctgaattcattcctcaaaacggttgtgcctctcctaagaattcaccagtagtaatactaataataaagacaatatgaacaatagctaatatgtattaagcataggctacataccagatactcttccaaggatatgatgcatactaaatccatctaatctctgtaacagcattattagttaccatcagcatttgaaacatcatgtccagaagagataagcattttgctcaccatcctacaggtagtatggaggtgaaatggtgatgacagtatggtatttgccatggataagggttttcctacatttgttacattaacagagttactctctaggatgaacttactgaagtttaacaaagactgaatagtgttggaaggcttctgcacatttaacatatctggtataaattatcttatgctgttacaggcattagaaaattttgattccctcatttgccaaatcttgctatagtatgaatattctgctattctaatcagagaggtgcaagtgaagaatttcttatttaaattgtcacttgtctcatgtcttgaaaagtgtgagtcttgtctcaaattatttctgggaaagaacaaactttgttttcaattctcaatcatttatggactgataattttgtaaaacagaatgttatggaaatgtcaaattgctataaaagttccaaatatttactcactttccacgtttatctcacaattgacagatgacaattttatgactgcaccagtctctggataataatttgggtagcatttgtctaaaggccttcctataattctaattcaaatgatttctcatttggatgaattctctgatgtactctaagatatttactgtgtctataagccttcccaaattccttatgtgcataggattacacagcagtatgaattctctgatgtgcagcaagaactgaattaagtttaggtccttcccacattcctcctatttaaactctttttaacaaataccaattatttgatgttaatcagaccttatgtcatgaatgaagatcttcacacattccttacatttaaatgattttacatcagtataaattgatatccaataagactgtacagaagtctaaaggccttttcatattaattatattcaaaatatttctcactagtatgaattgctggatagcaagataattgcccataaacagaaatgaatggcttttgcacaacccttacattcacaaggtttctcaagagtaagagttcttattatgataagttgtctatacacacacacaaaatattcttttacaactttcaatcataaggtttcatcagtatcaattttctcatttgagtaagttgtccacagaaaggcttccccacattcgttatatttgtagggtttatcattactatgagttctctcatgaacaagttttgagccacaagtaaaggtcttcccgaattccttacgttgataaagcttctcaccagtatgaaatctctgatgaacactaagttgatagccactaccaaaggccttcccacagtctttacattcataagacttctcattagtatggactctctcatgcttaactaggcttgaaccccaactgaaggccttcccacattccttacatttgaaaggtttctcaccggtatgaattttctgatgttgagtaaggtgatagccacgactaaaagccttcccacattctttacattcatagggtttctcccctgtatggattctttcatgttgaacaaggcttgatccacaattaaaagccttcccacattccttacattcatagggtttctcaccagtgtgaaatacctgatgtcgagtaagttgatacccactacaaaaggtctttccgcattctttacattcatgggatttctcaccagtatgaactctctcatgtttaacaaggcttgaaccccaactaaaggccttcccacattccttacattcaaaaggtttctcaccagtatggattttctgatgttgagaaaggtgatagccacgactaaaggcctttccacattctttacattcataaggtttctcaccagtatgaattctttcatgttgaataagacttgatccgcaattaaaagccttcccacattccttgcattcatagggtttctcaccagtatgaaatatctgatgtcgagtaagttgatagccccaacaaaaagcctttccacatattttacattcataaggtttcttaccagtatggattttctgatgctgagtaagctgatagccacgactgaaggccttcccacattctttacatttataaggtttctcacctgtatgaattatctcatgtttagcaaggcttgagccccaaaaaaaggccttcccacattccttacatttataagatttcacaccagtatgaattttctgatgttgggtaaggtgatagccacgactaaaggccttcccacattctttacattcatagggtttctcaccagtgtgaattctctcatgtttaacaaggcttgatccccagctaaaggtcttcccacattccttacactcatagggtttctcaccagtatgaaatctctgatgcacattgagttgataggcacttaaataattcttcccacattctttacattcaaagtgtttttcagctgtatgagttctctcatgttgaacaagttttgagccatgactgcaagccttcccacattccttacaaacataggatttctctgtattatgaattctttgatgtggagtaagagatttactttttctgtaagaaggtattttttcatagctgattatcatttgactgaagtatccctcttgatgtccttttagtccctcgaatatgcttttgcacttccaattatttctgaagatggatgcctcaaggccaagggttttacttttgtccttcatctcccactgggaaaaatttatttcaaaaatatcattttctgaaaatatttttttggtctcatacgtttttgactccaaatccagtgacaccaagttactatagttctccaacattacatccacgtacaagtccctctgagcagggtccaggcattcccactcctcctgagagaagtcgatggccacatccctgaatgtcaccaacccatcagtcatggttctggaattgcaagaactaattaatgctccatgggattcctctattggtgaagcacagaatccagaaaagccagaactgtagtcccagctactcaggaggctgaggcaggagaatagcgtgaacccaggaggcggagcttgcagtgagccaagatcgcaccactgcactccagcctgggcgacagagcgagactccatcagctctcgaacatcctgtagctgttattcaatgtaatgagacacattcactgtcaagattctcctgaaccttgatttctaaacatgcaaaaatccttttctcctcttcaaactccttcttagaaatctggcaacctggcagcacatgcagagtccaagaaccttaaggacaccggaaaaggacccagagacctgtggttagtttggacccagaggctgatgggaaacaagagcctggaaatgctcgcaggctgggagaggagcttct

SEQ ID NO: 14339 - RNA, 5330 nt, Homo sapiens
  source 1..5330: mol_type = other RNA
gctgggattacaggcatgagccaccgcgcccggccgtctttttttttttttcacttctctttagtcttttgataagctggtgaggtgcttttgcttgttccttaggaggggatttagtagatgctactttataagcttctttaactgtaaaatcctccttcattgtcaagtactagtaagcactggtgattccttgagatataatttcagaaatgttgggataaggcaccatgtctacatttcttggttaacaggcaaatgtggcacccagagggagtggcataatagccagttaccaataatatatcctgttaaaactcccaaagtactctgctttgtgttacagttgattattaagagtgcaactgttggctttttatgcctttgaaaaagtgcaatcatgtagaatgatgatcactagatggtgaatgactgactgaacagtgatattacgaatcccctatgtgcacaaaatagagaggtcaggtgtagacctatgacaaggaaccacagacatttagttatcaatgcattagttctgatggaactgacattattttcaaaaagaaataatttttaaaagggtcgatttctaactgtgtgagtatataaacacacactctatttcttcataactaacctgccttgatgctagcactaaatcatgacaggcacctggttgaaagtggttgcaagaagccatcaattttaagatgcattgtgatttccaaatagtaaaatatagccaggcgcagtgtctcacacctgtaatcccaacactttgggaggctgaggcaggtgcaggagttcaagatcagcctggaccaacatggcaaaaccccatctctactaaaaatacaagaattagccagtatggtggtgcacacctgtgtatccagctacttgggaggctgaggcacgagaatcacttgaacccgagaggtgcaggttgcagtgagccgaaatcacaccactgcactccagccttggtgacagaaagagagatcctgtcccaaaaaaaaaaaaaagtaaaatacataccatatgatcacacatttccaaagatcattgatcaaggctgaccaatcctattaggtatataatggatctttataacagacaactccagtagttaccataagtgatcaaacttggcactggtgatactgggggaaatggatactatctgcttctgaggtattgcaagatgaagtacacatcaccatctatgaagtgttctggtaaaaaatgtttaagcctctatttccaacttcatgttacgagaaatgtgaaggagaggcccatatcaaatttcaccatgaggaatgaaactaatgtgtgacattctataaaacagctttcctaaactcttcaaaagtctggattttttcaagtctcatttttttagctcagcttaagggataaactctgaattaaaatcccctcaaattctttatactgtactagatcttatccagaatgaactatctgaaattcaaatggatgagtggttatgggaagcttttctgaattcattcctcaaaacggttgtgcctctcctaagaattcaccagtagtaatactaataataaagacaatatgaacaatagctaatatgtattaagcataggctacataccagatactcttccaaggatatgatgcatactaaatccatctaatctctgtaacagcattattagttaccatcagcatttgaaacatcatgtccagaagagataagcattttgctcaccatcctacaggtagtatggaggtgaaatggtgatgacagtatggtatttgccatggataagggttttcctacatttgttacattaacagagttactctctaggatgaacttactgaagtttaacaaagactgaatagtgttggaaggcttctgcacatttaacatatctggtataaattatcttatgctgttacaggcattagaaaattttgattccctcatttgccaaatcttgctatagtatgaatattctgctattctaatcagagaggtgcaagtgaagaatttcttatttaaattgtcacttgtctcatgtcttgaaaagtgtgagtcttgtctcaaattatttctgggaaagaacaaactttgttttcaattctcaatcatttatggactgataattttgtaaaacagaatgttatggaaatgtcaaattgctataaaagttccaaatatttactcactttccacgtttatctcacaattgacagatgacaattttatgactgcaccagtctctggataataatttgggtagcatttgtctaaaggccttcctataattctaattcaaatgatttctcatttggatgaattctctgatgtactctaagatatttactgtgtctataagccttcccaaattccttatgtgcataggattacacagcagtatgaattctctgatgtgcagcaagaactgaattaagtttaggtccttcccacattcctcctatttaaactctttttaacaaataccaattatttgatgttaatcagaccttatgtcatgaatgaagatcttcacacattccttacatttaaatgattttacatcagtataaattgatatccaataagactgtacagaagtctaaaggccttttcatattaattatattcaaaatatttctcactagtatgaattgctggatagcaagataattgcccataaacagaaatgaatggcttttgcacaacccttacattcacaaggtttctcaagagtaagagttcttattatgataagttgtctatacacacacacaaaatattcttttacaactttcaatcataaggtttcatcagtatcaattttctcatttgagtaagttgtccacagaaaggcttccccacattcgttatatttgtagggtttatcattactatgagttctctcatgaacaagttttgagccacaagtaaaggtcttcccgaattccttacgttgataaagcttctcaccagtatgaaatctctgatgaacactaagttgatagccactaccaaaggccttcccacagtctttacattcataagacttctcattagtatggactctctcatgcttaactaggcttgaaccccaactgaaggccttcccacattccttacatttgaaaggtttctcaccggtatgaattttctgatgttgagtaaggtgatagccacgactaaaagccttcccacattctttacattcatagggtttctcccctgtatggattctttcatgttgaacaaggcttgatccacaattaaaagccttcccacattccttacattcatagggtttctcaccagtgtgaaatacctgatgtcgagtaagttgatacccactacaaaaggtctttccgcattctttacattcatgggatttctcaccagtatgaactctctcatgtttaacaaggcttgaaccccaactaaaggccttcccacattccttacattcaaaaggtttctcaccagtatggattttctgatgttgagaaaggtgatagccacgactaaaggcctttccacattctttacattcataaggtttctcaccagtatgaattctttcatgttgaataagacttgatccgcaattaaaagccttcccacattccttgcattcatagggtttctcaccagtatgaaatatctgatgtcgagtaagttgatagccccaacaaaaagcctttccacatattttacattcataaggtttcttaccagtatggattttctgatgctgagtaagctgatagccacgactgaaggccttcccacattctttacatttataaggtttctcacctgtatgaattatctcatgtttagcaaggcttgagccccaaaaaaaggccttcccacattccttacatttataagatttcacaccagtatgaattttctgatgttgggtaaggtgatagccacgactaaaggccttcccacattctttacattcatagggtttctcaccagtgtgaattctctcatgtttaacaaggcttgatccccagctaaaggtcttcccacattccttacactcatagggtttctcaccagtatgaaatctctgatgcacattgagttgataggcacttaaataattcttcccacattctttacattcaaagtgtttttcagctgtatgagttctctcatgttgaacaagttttgagccatgactgcaagccttcccacattccttacaaacataggatttctctgtattatgaattctttgatgtggagtaagagatttactttttctgtaagaaggtattttttcatagctgattatcatttgactgaagtatccctcttgatgtccttttagtccctcgaatatgcttttgcacttccaattatttctgaagatggatgcctcaaggccaagggttttacttttgtccttcatctcccactgggaaaaatttatttcaaaaatatcattttctgaaaatatttttttggtctcatacgtttttgactccaaatccagtgacaccaagttactatagttctccaacattacatccacgtacaagtccctctgagcagggtccaggcattcccactcctcctgagagaagtcgatggccacatccctgaatgtcaccaacccatcagtcatggttctggaattgcaagaactaattaatgctccatgggattcctctattggtgaagcacagaatccagaaaagccagaactgtagtcccagctactcaggaggctgaggcaggagaatagcgtgaacccaggaggcggagcttgcagtgagccaagatcgcaccactgcactccagcctgggcgacagagcgagactccatcagctctcgaacatcctgtagctgttattcaatgtaatgagacacattcactgtcaagattctcctgaaccttgatttctaaacatgcaaaaatccttttctcctcttcaaactccttcttagaaatctggcaacctggcagcactctagaacttccccatcaggtcttgacaagatcctgtcccgcggacacttccagatctaaaattctcatccttcttgcttgaaacgttcattatggggcttagcatagacttctttcttgcggtcatttaattgtggcaggcccgaagacaggctaaagggaaccatgcagagtccaagaaccttaaggacaccggaaaaggacccagagacctgtggttagtttggacccagaggctgatgggaaacaagagcctggaaatgctcgcaggctgggagaggagcttctggcaggcaagctcgccccgcccctaaaag

SEQ ID NO: 14340 - RNA, 5055 nt, Homo sapiens
  source 1..5055: mol_type = other RNA
gctgggattacaggcatgagccaccgcgcccggccgtctttttttttttttcacttctctttagtcttttgataagctggtgaggtgcttttgcttgttccttaggaggggatttagtagatgctactttataagcttctttaactgtaaaatcctccttcattgtcaagtactagtaagcactggtgattccttgagatataatttcagaaatgttgggataaggcaccatgtctacatttcttggttaacaggcaaatgtggcacccagagggagtggcataatagccagttaccaataatatatcctgttaaaactcccaaagtactctgctttgtgttacagttgattattaagagtgcaactgttggctttttatgcctttgaaaaagtgcaatcatgtagaatgatgatcactagatggtgaatgactgactgaacagtgatattacgaatcccctatgtgcacaaaatagagaggtcaggtgtagacctatgacaaggaaccacagacatttagttatcaatgcattagttctgatggaactgacattattttcaaaaagaaataatttttaaaagggtcgatttctaactgtgtgagtatataaacacacactctatttcttcataactaacctgccttgatgctagcactaaatcatgacaggcacctggttgaaagtggttgcaagaagccatcaattttaagatgcattgtgatttccaaatagtaaaatatagccaggcgcagtgtctcacacctgtaatcccaacactttgggaggctgaggcaggtgcaggagttcaagatcagcctggaccaacatggcaaaaccccatctctactaaaaatacaagaattagccagtatggtggtgcacacctgtgtatccagctacttgggaggctgaggcacgagaatcacttgaacccgagaggtgcaggttgcagtgagccgaaatcacaccactgcactccagccttggtgacagaaagagagatcctgtcccaaaaaaaaaaaaaagtaaaatacataccatatgatcacacatttccaaagatcattgatcaaggctgaccaatcctattaggtatataatggatctttataacagacaactccagtagttaccataagtgatcaaacttggcactggtgatactgggggaaatggatactatctgcttctgaggtattgcaagatgaagtacacatcaccatctatgaagtgttctggtaaaaaatgtttaagcctctatttccaacttcatgttacgagaaatgtgaaggagaggcccatatcaaatttcaccatgaggaatgaaactaatgtgtgacattctataaaacagctttcctaaactcttcaaaagtctggattttttcaagtctcatttttttagctcagcttaagggataaactctgaattaaaatcccctcaaattctttatactgtactagatcttatccagaatgaactatctgaaattcaaatggatgagtggttatgggaagcttttctgaattcattcctcaaaacggttgtgcctctcctaagaattcaccagtagtaatactaataataaagacaatatgaacaatagctaatatgtattaagcataggctacataccagatactcttccaaggatatgatgcatactaaatccatctaatctctgtaacagcattattagttaccatcagcatttgaaacatcatgtccagaagagataagcattttgctcaccatcctacaggtagtatggaggtgaaatggtgatgacagtatggtatttgccatggataagggttttcctacatttgttacattaacagagttactctctaggatgaacttactgaagtttaacaaagactgaatagtgttggaaggcttctgcacatttaacatatctggtataaattatcttatgctgttacaggcattagaaaattttgattccctcatttgccaaatcttgctatagtatgaatattctgctattctaatcagagaggtgcaagtgaagaatttcttatttaaattgtcacttgtctcatgtcttgaaaagtgtgagtcttgtctcaaattatttctgggaaagaacaaactttgttttcaattctcaatcatttatggactgataattttgtaaaacagaatgttatggaaatgtcaaattgctataaaagttccaaatatttactcactttccacgtttatctcacaattgacagatgacaattttatgactgcaccagtctctggataataatttgggtagcatttgtctaaaggccttcctataattctaattcaaatgatttctcatttggatgaattctctgatgtactctaagatatttactgtgtctataagccttcccaaattccttatgtgcataggattacacagcagtatgaattctctgatgtgcagcaagaactgaattaagtttaggtccttcccacattcctcctatttaaactctttttaacaaataccaattatttgatgttaatcagaccttatgtcatgaatgaagatcttcacacattccttacatttaaatgattttacatcagtataaattgatatccaataagactgtacagaagtctaaaggccttttcatattaattatattcaaaatatttctcactagtatgaattgctggatagcaagataattgcccataaacagaaatgaatggcttttgcacaacccttacattcacaaggtttctcaagagtaagagttcttattatgataagttgtctatacacacacacaaaatattcttttacaactttcaatcataaggtttcatcagtatcaattttctcatttgagtaagttgtccacagaaaggcttccccacattcgttatatttgtagggtttatcattactatgagttctctcatgaacaagttttgagccacaagtaaaggtcttcccgaattccttacgttgataaagcttctcaccagtatgaaatctctgatgaacactaagttgatagccactaccaaaggccttcccacagtctttacattcataagacttctcattagtatggactctctcatgcttaactaggcttgaaccccaactgaaggccttcccacattccttacatttgaaaggtttctcaccggtatgaattttctgatgttgagtaaggtgatagccacgactaaaagccttcccacattctttacattcatagggtttctcccctgtatggattctttcatgttgaacaaggcttgatccacaattaaaagccttcccacattccttacattcatagggtttctcaccagtgtgaaatacctgatgtcgagtaagttgatacccactacaaaaggtctttccgcattctttacattcatgggatttctcaccagtatgaactctctcatgtttaacaaggcttgaaccccaactaaaggccttcccacattccttacattcaaaaggtttctcaccagtatggattttctgatgttgagaaaggtgatagccacgactaaaggcctttccacattctttacattcataaggtttctcaccagtatgaattctttcatgttgaataagacttgatccgcaattaaaagccttcccacattccttgcattcatagggtttctcaccagtatgaaatatctgatgtcgagtaagttgatagccccaacaaaaagcctttccacatattttacattcataaggtttcttaccagtatggattttctgatgctgagtaagctgatagccacgactgaaggccttcccacattctttacatttataaggtttctcacctgtatgaattatctcatgtttagcaaggcttgagccccaaaaaaaggccttcccacattccttacatttataagatttcacaccagtatgaattttctgatgttgggtaaggtgatagccacgactaaaggccttcccacattctttacattcatagggtttctcaccagtgtgaattctctcatgtttaacaaggcttgatccccagctaaaggtcttcccacattccttacactcatagggtttctcaccagtatgaaatctctgatgcacattgagttgataggcacttaaataattcttcccacattctttacattcaaagtgtttttcagctgtatgagttctctcatgttgaacaagttttgagccatgactgcaagccttcccacattccttacaaacataggatttctctgtattatgaattctttgatgtggagtaagagatttactttttctgtaagaaggtattttttcatagctgattatcatttgactgaagtatccctcttgatgtccttttagtccctcgaatatgcttttgcacttccaattatttctgaagatggatgcctcaaggccaagggttttacttttgtccttcatctcccactgggaaaaatttatttcaaaaatatcattttctgaaaatatttttttggtctcatacgtttttgactccaaatccagtgacaccaagttactatagttctccaacattacatccacgtacaagtccctctgagcagggtccaggcattcccactcctcctgagagaagtcgatggccacatccctgaatgtcaccaacccatcagtcatggttctggaattgcaagaactaattaatgctccatgggattcctctattggtgaagcacagaatccagaaaagccagaactgtagtcccagctactcaggaggctgaggcaggagaatagcgtgaacccaggaggcggagcttgcagtgagccaagatcgcaccactgcactccagcctgggcgacagagcgagactccatcagctctcgaacatcctgtagctgttattcaatgtaatgagacacattcactgtcaagattctcctggaagctcgtcaatggaacaagaagacctcaggttaagacttcctgtcgtaaggctgggcacagtggctcacgcctgtaatcctagcacttgaggagcccgaggcaggcagatcacttgag

SEQ ID NO: 14341 - RNA, 5201 nt, Homo sapiens
  source 1..5201: mol_type = other RNA
gctgggattacaggcatgagccaccgcgcccggccgtctttttttttttttcacttctctttagtcttttgataagctggtgaggtgcttttgcttgttccttaggaggggatttagtagatgctactttataagcttctttaactgtaaaatcctccttcattgtcaagtactagtaagcactggtgattccttgagatataatttcagaaatgttgggataaggcaccatgtctacatttcttggttaacaggcaaatgtggcacccagagggagtggcataatagccagttaccaataatatatcctgttaaaactcccaaagtactctgctttgtgttacagttgattattaagagtgcaactgttggctttttatgcctttgaaaaagtgcaatcatgtagaatgatgatcactagatggtgaatgactgactgaacagtgatattacgaatcccctatgtgcacaaaatagagaggtcaggtgtagacctatgacaaggaaccacagacatttagttatcaatgcattagttctgatggaactgacattattttcaaaaagaaataatttttaaaagggtcgatttctaactgtgtgagtatataaacacacactctatttcttcataactaacctgccttgatgctagcactaaatcatgacaggcacctggttgaaagtggttgcaagaagccatcaattttaagatgcattgtgatttccaaatagtaaaatatagccaggcgcagtgtctcacacctgtaatcccaacactttgggaggctgaggcaggtgcaggagttcaagatcagcctggaccaacatggcaaaaccccatctctactaaaaatacaagaattagccagtatggtggtgcacacctgtgtatccagctacttgggaggctgaggcacgagaatcacttgaacccgagaggtgcaggttgcagtgagccgaaatcacaccactgcactccagccttggtgacagaaagagagatcctgtcccaaaaaaaaaaaaaagtaaaatacataccatatgatcacacatttccaaagatcattgatcaaggctgaccaatcctattaggtatataatggatctttataacagacaactccagtagttaccataagtgatcaaacttggcactggtgatactgggggaaatggatactatctgcttctgaggtattgcaagatgaagtacacatcaccatctatgaagtgttctggtaaaaaatgtttaagcctctatttccaacttcatgttacgagaaatgtgaaggagaggcccatatcaaatttcaccatgaggaatgaaactaatgtgtgacattctataaaacagctttcctaaactcttcaaaagtctggattttttcaagtctcatttttttagctcagcttaagggataaactctgaattaaaatcccctcaaattctttatactgtactagatcttatccagaatgaactatctgaaattcaaatggatgagtggttatgggaagcttttctgaattcattcctcaaaacggttgtgcctctcctaagaattcaccagtagtaatactaataataaagacaatatgaacaatagctaatatgtattaagcataggctacataccagatactcttccaaggatatgatgcatactaaatccatctaatctctgtaacagcattattagttaccatcagcatttgaaacatcatgtccagaagagataagcattttgctcaccatcctacaggtagtatggaggtgaaatggtgatgacagtatggtatttgccatggataagggttttcctacatttgttacattaacagagttactctctaggatgaacttactgaagtttaacaaagactgaatagtgttggaaggcttctgcacatttaacatatctggtataaattatcttatgctgttacaggcattagaaaattttgattccctcatttgccaaatcttgctatagtatgaatattctgctattctaatcagagaggtgcaagtgaagaatttcttatttaaattgtcacttgtctcatgtcttgaaaagtgtgagtcttgtctcaaattatttctgggaaagaacaaactttgttttcaattctcaatcatttatggactgataattttgtaaaacagaatgttatggaaatgtcaaattgctataaaagttccaaatatttactcactttccacgtttatctcacaattgacagatgacaattttatgactgcaccagtctctggataataatttgggtagcatttgtctaaaggccttcctataattctaattcaaatgatttctcatttggatgaattctctgatgtactctaagatatttactgtgtctataagccttcccaaattccttatgtgcataggattacacagcagtatgaattctctgatgtgcagcaagaactgaattaagtttaggtccttcccacattcctcctatttaaactctttttaacaaataccaattatttgatgttaatcagaccttatgtcatgaatgaagatcttcacacattccttacatttaaatgattttacatcagtataaattgatatccaataagactgtacagaagtctaaaggccttttcatattaattatattcaaaatatttctcactagtatgaattgctggatagcaagataattgcccataaacagaaatgaatggcttttgcacaacccttacattcacaaggtttctcaagagtaagagttcttattatgataagttgtctatacacacacacaaaatattcttttacaactttcaatcataaggtttcatcagtatcaattttctcatttgagtaagttgtccacagaaaggcttccccacattcgttatatttgtagggtttatcattactatgagttctctcatgaacaagttttgagccacaagtaaaggtcttcccgaattccttacgttgataaagcttctcaccagtatgaaatctctgatgaacactaagttgatagccactaccaaaggccttcccacagtctttacattcataagacttctcattagtatggactctctcatgcttaactaggcttgaaccccaactgaaggccttcccacattccttacatttgaaaggtttctcaccggtatgaattttctgatgttgagtaaggtgatagccacgactaaaagccttcccacattctttacattcatagggtttctcccctgtatggattctttcatgttgaacaaggcttgatccacaattaaaagccttcccacattccttacattcatagggtttctcaccagtgtgaaatacctgatgtcgagtaagttgatacccactacaaaaggtctttccgcattctttacattcatgggatttctcaccagtatgaactctctcatgtttaacaaggcttgaaccccaactaaaggccttcccacattccttacattcaaaaggtttctcaccagtatggattttctgatgttgagaaaggtgatagccacgactaaaggcctttccacattctttacattcataaggtttctcaccagtatgaattctttcatgttgaataagacttgatccgcaattaaaagccttcccacattccttgcattcatagggtttctcaccagtatgaaatatctgatgtcgagtaagttgatagccccaacaaaaagcctttccacatattttacattcataaggtttcttaccagtatggattttctgatgctgagtaagctgatagccacgactgaaggccttcccacattctttacatttataaggtttctcacctgtatgaattatctcatgtttagcaaggcttgagccccaaaaaaaggccttcccacattccttacatttataagatttcacaccagtatgaattttctgatgttgggtaaggtgatagccacgactaaaggccttcccacattctttacattcatagggtttctcaccagtgtgaattctctcatgtttaacaaggcttgatccccagctaaaggtcttcccacattccttacactcatagggtttctcaccagtatgaaatctctgatgcacattgagttgataggcacttaaataattcttcccacattctttacattcaaagtgtttttcagctgtatgagttctctcatgttgaacaagttttgagccatgactgcaagccttcccacattccttacaaacataggatttctctgtattatgaattctttgatgtggagtaagagatttactttttctgtaagaaggtattttttcatagctgattatcatttgactgaagtatccctcttgatgtccttttagtccctcgaatatgcttttgcacttccaattatttctgaagatggatgcctcaaggccaagggttttacttttgtccttcatctcccactgggaaaaatttatttcaaaaatatcattttctgaaaatatttttttggtctcatacgtttttgactccaaatccagtgacaccaagttactatagttctccaacattacatccacgtacaagtccctctgagcagggtccaggcattcccactcctcctgagagaagtcgatggccacatccctgaatgtcaccaacccatcagtcatggttctggaattgcaagaactaattaatgctccatgggattcctctattggtgaagcacagaatccagaaaagccagaactgtagtcccagctactcaggaggctgaggcaggagaatagcgtgaacccaggaggcggagcttgcagtgagccaagatcgcaccactgcactccagcctgggcgacagagcgagactccatcagctctcgaacatcctgtagctgttattcaatgtaatgagacacattcactgtcaagattctcctgtagtcccaggtactcgggagcctgaggtgggaggatcgcttgagcctaggaggccaaggctacagtgagccatgatcatgccactgcactccagcctaggcaaaaggccaagaacctgaaccttgatttctaaacatgcaaaaatccttttctcctcttcaaactccttcttagaaatctggcaacctggcagcacatgcagagtccaagaaccttaaggacaccggaaaaggacccagagacctgtggttagtttggacccagag

SEQ ID NO: 14342 - RNA, 13893 nt, Homo sapiens
  source 1..13893: mol_type = other RNA
gctgggattacaggcatgagccaccgcgcccggccgtctttttttttttttcacttctctttagtcttttgataagctggtgaggtgcttttgcttgttccttaggaggggatttagtagatgctactttataagcttctttaactgtaaaatcctccttcattgtcaagtactagtaagcactggtgattccttgagatataatttcagaaatgttgggataaggcaccatgtctacatttcttggttaacaggcaaatgtggcacccagagggagtggcataatagccagttaccaataatatatcctgttaaaactcccaaagtactctgctttgtgttacagttgattattaagagtgcaactgttggctttttatgcctttgaaaaagtgcaatcatgtagaatgatgatcactagatggtgaatgactgactgaacagtgatattacgaatcccctatgtgcacaaaatagagaggtcaggtgtagacctatgacaaggaaccacagacatttagttatcaatgcattagttctgatggaactgacattattttcaaaaagaaataatttttaaaagggtcgatttctaactgtgtgagtatataaacacacactctatttcttcataactaacctgccttgatgctagcactaaatcatgacaggcacctggttgaaagtggttgcaagaagccatcaattttaagatgcattgtgatttccaaatagtaaaatatagccaggcgcagtgtctcacacctgtaatcccaacactttgggaggctgaggcaggtgcaggagttcaagatcagcctggaccaacatggcaaaaccccatctctactaaaaatacaagaattagccagtatggtggtgcacacctgtgtatccagctacttgggaggctgaggcacgagaatcacttgaacccgagaggtgcaggttgcagtgagccgaaatcacaccactgcactccagccttggtgacagaaagagagatcctgtcccaaaaaaaaaaaaaagtaaaatacataccatatgatcacacatttccaaagatcattgatcaaggctgaccaatcctattaggtatataatggatctttataacagacaactccagtagttaccataagtgatcaaacttggcactggtgatactgggggaaatggatactatctgcttctgaggtattgcaagatgaagtacacatcaccatctatgaagtgttctggtaaaaaatgtttaagcctctatttccaacttcatgttacgagaaatgtgaaggagaggcccatatcaaatttcaccatgaggaatgaaactaatgtgtgacattctataaaacagctttcctaaactcttcaaaagtctggattttttcaagtctcatttttttagctcagcttaagggataaactctgaattaaaatcccctcaaattctttatactgtactagatcttatccagaatgaactatctgaaattcaaatggatgagtggttatgggaagcttttctgaattcattcctcaaaacggttgtgcctctcctaagaattcaccagtagtaatactaataataaagacaatatgaacaatagctaatatgtattaagcataggctacataccagatactcttccaaggatatgatgcatactaaatccatctaatctctgtaacagcattattagttaccatcagcatttgaaacatcatgtccagaagagataagcattttgctcaccatcctacaggtagtatggaggtgaaatggtgatgacagtatggtatttgccatggataagggttttcctacatttgttacattaacagagttactctctaggatgaacttactgaagtttaacaaagactgaatagtgttggaaggcttctgcacatttaacatatctggtataaattatcttatgctgttacaggcattagaaaattttgattccctcatttgccaaatcttgctatagtatgaatattctgctattctaatcagagaggtgcaagtgaagaatttcttatttaaattgtcacttgtctcatgtcttgaaaagtgtgagtcttgtctcaaattatttctgggaaagaacaaactttgttttcaattctcaatcatttatggactgataattttgtaaaacagaatgttatggaaatgtcaaattgctataaaagttccaaatatttactcactttccacgtttatctcacaattgacagatgacaattttatgactgcaccagtctctggataataatttgggtagcatttgtctaaaggccttcctataattctaattcaaatgatttctcatttggatgaattctctgatgtactctaagatatttactgtgtctataagccttcccaaattccttatgtgcataggattacacagcagtatgaattctctgatgtgcagcaagaactgaattaagtttaggtccttcccacattcctcctatttaaactctttttaacaaataccaattatttgatgttaatcagaccttatgtcatgaatgaagatcttcacacattccttacatttaaatgattttacatcagtataaattgatatccaataagactgtacagaagtctaaaggccttttcatattaattatattcaaaatatttctcactagtatgaattgctggatagcaagataattgcccataaacagaaatgaatggcttttgcacaacccttacattcacaaggtttctcaagagtaagagttcttattatgataagttgtctatacacacacacaaaatattcttttacaactttcaatcataaggtttcatcagtatcaattttctcatttgagtaagttgtccacagaaaggcttccccacattcgttatatttgtagggtttatcattactatgagttctctcatgaacaagttttgagccacaagtaaaggtcttcccgaattccttacgttgataaagcttctcaccagtatgaaatctctgatgaacactaagttgatagccactaccaaaggccttcccacagtctttacattcataagacttctcattagtatggactctctcatgcttaactaggcttgaaccccaactgaaggccttcccacattccttacatttgaaaggtttctcaccggtatgaattttctgatgttgagtaaggtgatagccacgactaaaagccttcccacattctttacattcatagggtttctcccctgtatggattctttcatgttgaacaaggcttgatccacaattaaaagccttcccacattccttacattcatagggtttctcaccagtgtgaaatacctgatgtcgagtaagttgatacccactacaaaaggtctttccgcattctttacattcatgggatttctcaccagtatgaactctctcatgtttaacaaggcttgaaccccaactaaaggccttcccacattccttacattcaaaaggtttctcaccagtatggattttctgatgttgagaaaggtgatagccacgactaaaggcctttccacattctttacattcataaggtttctcaccagtatgaattctttcatgttgaataagacttgatccgcaattaaaagccttcccacattccttgcattcatagggtttctcaccagtatgaaatatctgatgtcgagtaagttgatagccccaacaaaaagcctttccacatattttacattcataaggtttcttaccagtatggattttctgatgctgagtaagctgatagccacgactgaaggccttcccacattctttacatttataaggtttctcacctgtatgaattatctcatgtttagcaaggcttgagccccaaaaaaaggccttcccacattccttacatttataagatttcacaccagtatgaattttctgatgttgggtaaggtgatagccacgactaaaggccttcccacattctttacattcatagggtttctcaccagtgtgaattctctcatgtttaacaaggcttgatccccagctaaaggtcttcccacattccttacactcatagggtttctcaccagtatgaaatctctgatgcacattgagttgataggcacttaaataattcttcccacattctttacattcaaagtgtttttcagctgtatgagttctctcatgttgaacaagttttgagccatgactgcaagccttcccacattccttacaaacataggatttctctgtattatgaattctttgatgtggagtaagagatttactttttctgtaagaaggtattttttcatagctgattatcatttgactgaagtatccctcttgatgtccttttagtccctcgaatatgcttttgcacttccaattatttctgaagatggatgcctcaaggccaagggttttacttttgtccttcatctcccactgggaaaaatttatttcaaaaatatcattttctgaaaatatttttttggtctcatacgtttttgactccaaattgaactcactccttggcattaaggcactcccttgttaaataacaaactcagccttgattttgcagctcttgtgatctgaatgttctgattttatagttttctggaggattccacagaggtcgcttcaacaagtccctcattttcccacgctgatgttccctcaaaccaaatgtcagcttccatcaatcaagcccttatgtgcccagttgtggtcatccaatgtatcttaatgggaatcaaattcttatcataatgagctttggctgattttgttttgtctaacaactcttttgtctaacaactcaatggtcgcaactctgccattttatcaaggcagccatgggcaatatgtaaacatataaacaaatgggcaagactatgttccaatacaactttatttgcaaaaacaggtggatttggcctccagagccagagttttccaacccctgagataaagcaaacattgctttcataaatgttcacaattgtaaaaatataaagttcaattaaattttacatttacttagatttattagccagaatttttataaaaggattgatttttataacttcatataatgctgcaattatgtgactctatagattttaccttatttaaaaattttaaatgtctatcaattttaaaaatcaacagtaattgtattgctatttaaggatcactttaaattataagatctccaattcacttagacaaaatgatcttgagagttactaataaataatttctggttgcataaaaagttcctaagaagatattcataaaagaggaagaacaaatattttgagttatttttcaattaagtttacttatttcttgaccattgttaaacatattttcactcaactaagctcaaactaccctgtcaaaaatcaatgtgatacacacatcatcttataacacattaatactgttaattatattttaaaattgaaaataaagctttaaattatagtgtcattcagcatggtatattgacaatattagcaggtttaaatgcatatgggaaatgctatgtcatataatgtatgaaaaaagtgacataagtatgatatgatagaaaagactgctagctaagggaaaatgatgatcttggagtaaactgtccactctatatgaggaaattaaagtattattctttttcttcaatacatgaagaaaataaatctgcataattttgccacacttctgtgtatgcttcaaattttaagagtcaaataattttcatgcttttagctaccttatactacacatctaaactatttttaaatagaacagaattttttatttaaataaaaattaaaatcttgctaccttctcattattttaaatattgtgttgatgttctgattaattagtcacaactattgttcttgtcaaaagctcctctgacaactctttttgttaatgccttttccaattcagaataatgaaacagattgtaacagattatgtctttcacataaaatctgcctttcaggtttcctaaaaggccactgagcaagcacaaagatttgctctttcgcttacaaaagatactagaaacaatcaggtttctttgacataatccagaatttacttagcccaaaactactatgactgtgtttttgtttatataaccccaggtatattaaaaaccaaaagctgacaataaaaagagaagtttggcctttctaggctaataagttacttgttattaaaaggtacctgtcccagcaataatgtacttgtcaagttggagaagatgtatattcatattcatgtacccacaggttatgactttctataaattaattttaagaaagattgtgtacctaggtttaaatacccttgtcaatttggaacaatcgtaatactctttcattgtccataatgtgttttgacttcaaggtagtcacttactttatccttataaattaattaggttttatacctcaatagaggatttaatttttttccattatgaagttgttgtttattatattaaattaaccagagccattgagccttaacaactacaagaaggtttttccaaactcaaatctactgacatttgggcccaaatcattcttggttgtgcggggttttcatgtgccttgcctgttgatgactgtataacattttggttgagctattaaatgatggatgattattgtgatgtgaatgtgggaagtaagtttaatcatatatagttggtcacaggtctaaactgcactattgctgtttcatttaacaatgtcttgctgctttttatgcattaacatttgggtgtaaagattctgtggataaccaaaacaaagccacagtatttaagctgaccaacctaatattccaactgaatatggaggtgaccaattatgaactaaaaggagtacagttttgtacaacatagcatcagtagtttagcgaattttaatttctatgtaaggcttagattttaatttaacattatagatttagatttaacattttagttacttactacttatgttttatgtaaggttttacagtgtcagtaaataaatatgggtttaacttcttaaatgtcaagaaaaatcattgaggacccaaaagacttttagtttatgtagttatatattttgatatttgtcatgttaaaaatttaaacagagaaattttaagatatttactaattcacttaaaataacaataaaccattaactgttaacataaatgatttgttataaaaataatcttttctaaaacaaaacaaaagatgttttaaattttttcaaatcttttaaatggatggtttaataaaagacacctggattctcatatctgcttctgcattcaatctatggcaatatgttatttaggttgaaatatatgaagaaaatcatatatatgaagtatatgaagaaaatctagcctctcatggtacatagttggaaaatggcagaatattttactagtccatgcagataactgtggatatttttctttgacaccaccctaaaacttaagaaatggtagtgtctggcaggttaagtacaatgtggaatataaaatcatatctgtgaacttttcatactatgttacattgcactttgaataatcttttatccatgtgtaattttgtaacatcatacactggtcatttggaaaatactgattcaaagagttatgcagatctttgaaatgttgacgtagttcactatacaacatcaaaaaatcacatgttaatattaccacccatctcataaaaaatcttaatgtattaggaagctataaagctcaaaattatgaataaacattttacaaaattctaattttaacatgacagattgaattatatcattggcaacaaatattagttatttttgaagtgacaggctcacttgcaagaaaatgttttcctactgcccaagtctgaacaaacaaagtttttcattctttggtgaaaaatatggtgttttgtcaaaaaagcagttggtttaactcacaatttttttgggggtggggacgtagtctcactttgtcaccaggctggaatgcagtggcacgatcttggctcactgcaacctccgcctctcgggttcaagcgattctcctgcctcagcctcccgagtagctgggactacaggcgcgtgccaccatgctcagctaatttttgtatttttagtagagatggggtttcaccatgttggccaggatggtctcgatctcttaaccttgtgatctgtccgccttggcctcccaaaatgctgggattacgggcatcagccacagagcctggcctttaactcacaacttaaacaactgtacaagtggttttcttcaaggcaaccatcatactttggtatacagcagaagaccttaatggatacttcccatttcattacatagaatattttttaaatgtatatataatcaagggttgagatttaataaaatgaatactgcttcttcaagatgttcttaagtgaaaatgggttttttcttaacacattttctttgtgtgtggaggtaaagaatatgatgattactagtactatttggtgcctctgcctttgctcatgctaaagcagagaagattcaccatggcttctacaccaccagtggaagtgtcaccacagtgaaaaaggcaaacctctcagtattgttatgagaatatttttcactttgtgaaaggtttggcccactgaaaggttcttgggaactcccaggggtcttcagtccacagtttgagaaccactgccctacctagagtaagaattatgtccaggactaaggataaaaccaaactgtacctgccttcaaaaatcaactcttaaaaagatcattgtgatctgctattaatttaactgcttgcctgaacagtttaactattaggaagataataaaatccccaagtcactacaacatggcatctacaatggccagtatacaatgagaaattgtaagaccggtaaagaagcaggaaaatttgacacaagatttagagaaaatacagtcaataaaagcagacccacaaaaccaaatgtaaattctataactataaaatgtaggtggaatgaaatctttattggataggcttaacaataattggacactatcaaagaaaaaaaaaacagtgacttcaagacaggtaaataggtattaccaaactgaagtacaaagagtaaaaagactgggggttgcacctccgtgactggtggcaccatataagtggtctaacacacatataattggagtcttaggaggaggaaaagtactaaagaagcagaaaaaagtatttgaagatacaatggttgaaatttctccaaattcaataaaaaaatcaacccactgatcaaaggtaagggaaagtgaagcatgataaatgtaaaggaaccatatctagaactttatagtcagattattacagaccaaaaataaagaaaaaacttaataacagagaataaagtatatataaaatgaacaataagaatcatagctgtctaatcattatatacaatagagttcagaagataatggaacatttttgaagctaactaaaagaaaaaatatatcagttgggaaattcatatctggtaaaaatatccttcaaaaataagaaagatgaaggctgggtgcagtggctcatgcctgtaatcccagcactttgggaggccaaggcaggtggatcacctgaggtcaggaaatcaaaaccagcctggccaacacagtgaaaccttgtgtctactaaaaatacaaaaactagtcaggcatagtggcacacgactgtaatcccagctattttggaggctgaggcacgagaattgcttgaacctgggaggcagaggctgcggtgagctgaaatcatggcactgcactccagcctgggtgacacagtgagactgtctcaaaaaaaaaaaaaaaaaagataaaattagctgctagtagccatataacacaagaaatgctaaaggaagcttttcaggctgaatgaagtttacagattagtaaaattcttacattatacaacaaagtagtatgttattaatttcaagtagaccatgctaaattaaggatgcatattgtaatcccaaaagtaaatacaaataatacagcaaaagataacagatgagataaaatggaatactaaaaaatacttgatgaatccaagaaggtggaaacaaaagaaagaactagtgaaacaaaaaatagcaagatagtaaactgaaatctaaccatatcaatagtgacattaaatgaatatgtaggagtgatgtcacacaaaatgatgaaataggaagctctaagggctggtacctccatcaaagcaacaattgagctggaaagacagattgtcattggccaggtgcggtgggccacacctgtaatcctagcattttgggaggccgaggtgggtggatcacgaggtcaggagattgagaccatcctggctaacacggtgaaacctcatctctactaaaaaataaaaaaaaaaaaggagaaaaaaaattagccgggcgtggtggcaggcgcctgtagtcccagctactcaggaggctgaggcaggagaatggtgtgaacctgggaggcagagcttgcagtgagccgagatcacaccactgcactccagcctgggtgacagagcaagactccatctcaaaaaaaaaaaagagagagagagattggcatccacaaactcttaattctggaatcttatcaggcacttccataacaacaaggggagtgctggatgaataaagaggctactattcttaggtgaaagagtggctcgtgcaagccaccatcccccatttctcagtccagccaatgctatgggatgacaggcctatgtgcctggaatgctgtgtaccaactaatcacttccttcactcctcagctccaccacagctgtggggagagcagcctgtattcctggaacagccggttgggacctgggtgggcagcgtgaccttgtcttccaaaaaattcagggttgtgcagtttggtgggttttgtgttaccttgagggaccagcacagataactgccttgattttagccccatcagccacagcagctttccccagaagtatctattggaagatttaaagggctaatggacctttttttcctcccctttttacagccagatatttaagtaaatctttgtctggtactaactgactgtagagatgatggaacagaaatttcagtgaccacatacaataaggaatatacaatttgcaaaaagagtttgaaaaaatctgacagctccagccctcaacaagcagaaatcagctatgcctgaggaatgggaaaattgaatctccagaggtaccacattataatactcaaaatgcccagttttaacaaaaaaaattacaaagcatacagtgaaacaggaaaatatggggcccgttcaaaggaaaaaaaagaatctgacagaaaccattcctgaggaagcccagacattaaatgaactatccaaatatgctcaatgagctacagaaaccatggaccaagagctaaaggaaatcaggaaaagaatgtatgaacaaaatgaaaatatcaataaaaggatagaaattataaaaaaaaggaaccaaacaaattctggagtaaagtaactgaaatgaaaatttcaatagtggattcagcagaagaaagactcagcaaacttgaaaatgagtcatttgaaattattgcactagagaagcaaaaagaaaaaggaataatgaacagtgaagagagcctgagggatcaatgggataccatcaagcacaccaacatacacatcatatgagtcccagaaaaagaagagagacaaaagtagagaaaaaaatttgaagaaaaaatgtctgaaaacttccaaaatctgacaaaaggcaggaatacacacatccaagaggctcaacaacttcagacatgataaagagattcatatctagacacattattgtcaaattatggaaacccaaagacaaaaagacttcagaacacaggaagaaagcagcagcctaccacatacaagaatctgcaacaagattaacagctaatttctcatcagaaaccacagagaacagaaagtaacaggatggtatattgaaaagtccaaaagaaaaaaaaaactgtcaaccaagaattctataccagcaaaaactgtcctttaagaataaaggtgaaattaaggcatttccagaaaaaacaaaagctgaaggaggtgattaccagtagacctactctagaagaaatgttagacaagagtgtttcagactaaagtgaaaggacactaaacagtaattagaagccataaggagaaataaagaacattggtaaaggtaactacatgagtaaatataaaagttagtattattgtacttttgatttattgatttaaaagacaaatgcataaaataataactataaatctgtgtgaaagtaaccaggcacttcaaagcaatagctgattgtaaaactagacaagggaaatttcatacaagatgaacctctaacaccttgtttatcagaaaaccaggaggtactcaaagagtgacggagatgtgccaaaaagccatatcatgaaaggattcccactgactaaatctggacaagctccaacactttgagcttcaaaataaataacagaaaaaaaacagaatatagcccattgactagaaagcgaacatatgaataaatggaaagtttaaagaggaacacaatatttatttatttattgaggtagggtcttgtgtgtcacccaggctggagtgtggtgacacaatctcagctcactgcagcctcaacctcttaggttcaagcaatccagccacctcagcctccccagttgctgggactaaaggagcgcaccaccacagcccagcaaatatttttgtattttttgtagagatggggttttgccatgctgcccatgctggtctcgaactcctggcctcaagtgatccaaccgtctcagcttcccaaagtgctgggattacaggtgtgagccaccactgtgcccagttccacaatatttaatagtttcaaagttcctccccacaaaatagttgtggaagggaaaaagggcaactgcacaaggaggaagccagcagacgctaccttaatcaagtactcagagtgaataacatgagtaatgataaattaatcataccacccaacaaaatgcagggagaagaacgcagcatcaattctgtgataatcctgccaaagatccatattctaaatctaatcatgaagaaatagcagacaaacccacattcaggaacactatacaaaatagctggcctgtaatcttcaaaagcatcacagacatatacgcaagtcaaggaaagacatgtgaactgtttcagactgaaagagactaaacaatccaaattccacaaacaagaacaacaaaacaatgtattatctggccccttcctatctccctggcctaatttcttagtacatgttcctttaataactctactctagagttctggtaaagttcctttccaacaacagggtctttgcatttgctgttcactgtgactgatctgttcctccgccagatattcacatagagatcccaggctccacatctctgttcaagaaagcgttccccgactgtcttacctaaattagccctgtcagtcctcatcattttctattcccttatgctgtttaccttttccaaagaatttgcttcattacatactatttatctatttataaatttacttatttgatgtttctgctttactacaaagtaaactgcacgaaaatgggcaagttatcaaagcttgttcatgattcaattgacagtgctcagcacaaggctggccaggagtagatattcaatataatatttgcagaatttatgaaat

SEQ ID NO: 14343 - RNA, 1710 nt, Homo sapiens
  source 1..1710: mol_type = other RNA
gctgggattacaggcatgagccaccgcgcccggcctaaaaatctgtagtaggaatattttatgcatcggctcgtttccagagagaagggagcatccgaggaagattcactgtgggttataataggaacctaaaaatagagctatgttgaatgtagcgatcataacatgttgctaataagactcttgaggttaacagctcaggtaagcatgtaagttcctgggaactcttagcgatgaaaatgatgtggagtggggaagagagtagaggaaccgagacacattaaagacactgcgcattcatttgagaatgctgatttcatgaaggtttaaaccaactgagtgtccctgggtgcagacattaaaactgcccagggatcaacctaggagtaaggatctgtcatcactcaccaacttagtcctgacaccatggccagctttggtgaccatctctgccatctcaagattgctgtgttttgctgaacggggagggccatccaggaattcaatgtcagattgtcaatcaaaaggcacttgtaggatgtcagtgcacttcctgtccttcagcttcttgcaaggatttttttttttatggagtagcgtggagttgctggattacggcaaacaggttgagtcgcagtgccaagtctgctgaacactgcttatctgaagggcatgtttgcagcactctgagtttgcagtagattacagcaccttccggcctctagcattagatgagaagaaaataaacaccaaagcttatagaacgcttctttcctcgaggctgcagaaggaaaccatttctctctttatggtagaaagcgtcctccatccaaagactgattccacaccttggcattttatccacctaaaaataaatagttgaaaaaggagaatatttctagcataaggaatatgtgaaagaatctgcctccctgggtgcagatattcctttttaacctgacatcctttttcaccaaaatccactgcttttaaactcaagatgaacagaatctcaaacccacactccccttgtaggaacctggcagagtgtctggcttgtcacatcccacttgtctgacgtatacctggattttctgttttgttttgttttgaaagtctacttctccaaaatgcctaatcttgatattttgaccctcatttgtctccccaaaccagtccttcatttgcctgcagacacagcccttctcatcagtccctttcatttcccactgacacttgctctcgatgctctttgcagaaaaaaaaaaaatgtgtgctgtgaacgcagtttgacatttcctgacatttcatgaactaattacactacaaataattaagcatgttcacatctgtaacaaacgaaggcaaaatggttgtcagcgggcgtgattgatgacttccctgagatttgatctgatgagattctccccatcgtgggcagaagcccgacgccacggtgtttgcaatcatgccttcagcccttttcatgagatcacaccgacgagatgagtggttccacttgtgatttttcaactctttgatggcatgaaagtgatctgcattcagtggaaagcgtaacttcatattgtaagttgagagctttatgtcagttttgacttcttttttgacgtatgatgggtttatccagatgtagcgccatcataagtcaaggagcataatcatggctgaaggggaaaaggcacttcttac

SEQ ID NO: 14344 - RNA, 7071 nt, Homo sapiens
  source 1..7071: mol_type = other RNA
gctgggattacaggcatgagccaccgcgcccggcctaaacgtgagacttttaatgacggtcttgcaagatcgggtgtctggtgggcaggcacacccagcacggtcacaacaagccatttatcccccagtacgcaggcccctcccccggttcctcacaggctgagtactctggggtcacagtcttcccggacatcacctattggttgtcgggcaggggctgtaggtgtttttttagggttgtcctgctgcattttgttgcagcccacaatgcgttgcaatcctagtcagctcaggggcttttcaggtatttgacttatgacctaagtagctgggcagactgataagaacagacaaaacaagctatgttgcagacgagtaaaactttcgtcatagactaaaagtttttgggtcaggtgaaggcaactaagcgttggggggaagactggggatggggaggccgacaagcaggcatcggcaacccaggcaggggcctggtcttctgtagcttgctgacctaagcaagcaagacactgtgtcttggaagtggaccactgtgtacattatttccttcactgagaactgattttgcaaagccgagtttgtgtgactgtggagggcgagtgtccacaccaggcagcgtccaactcagcgctgtttctcagactgatgtcccggggacagtcacagacccccggggctgtcctgctccctgccgggtggcagtgaccatggggatgtgcatgagggctctaggtctgaggggtggtttgtccaaggtcatggtcagagccaggactgacacctgggttccagcctccgtgccaggggtgtggcgtgagcaccacgaggggaaactggggacatgtgacacactgcagcgctgaggggccctgttctgaggagccagtggagaccgagtcgtgtcggccccatgccgcctattgagaggcatccgtgccggccgcgcagggctccctctggtccaggcgctctggtcctcggcggggcccctgctctcctggtggggccctgaaagtgacggcaccccgacggccactggagggagctccagaaccgagcctgcccttgaggccggaaaccgcggctggccctggagctgcctttggatcgcggagtattaaaagtgcccgcacttgaaatcttactgcgtgtcctgaagagagccctgtccctttcccatgagatgctgagccgtgatctgtactcgggaagcacacagatctcctgtctccaccctggcgtgttctgacaggtgcagccgctgtgtcaccagcaccccggcaagggagaccgcctccgtcgcccctccctggcccacgccctcccagacccggccctcgtcgccgctgtgtcgctggtgaggtgggttccctgctctggagctgctgaagaggctccagtactttgcacgtgctcacatctagctgtgtccccgcagctgcatgttttgtgaggttcaccctgttgccgcgcctgtccccggtgggtccatttcgctgacgagtagcattccttcgatgcgcaggccacatctgtttatctgtccacctgttgatgtgcagttgggttgtttccagtgttgggctcttatgagcaaagctgccgtgaacatttgtatacaggtgcttgtgtggacttccgttcccatttttcttgggtaaatgtctggaattgggacagcggggacagatgttaaccatgtttaattttggaagtggctgccaagtggggtacgttttaccttcctcccaccacctcagctgcacacttagtgtatgccagttggctggagctgggcaggaagccagcctgtccagccttgggtctggagaggggccccaaggggtgccgtggcccctagaacaggatggggccatgtttcctcctgcccagggcctcatcgtttctcagactggtgctgggaagaatcttcgtgccccaaggggctctgcagaaagcgtcctgtgatgattagggttggacagcggggaacgctgtcttttctctttagaagccttagtgtgtgtggcacagctcagatgtcctgcagaaaagaatcggatgctgctcgcttgacccggcgtttcccaccctccctcctggggccttctgtgcgccctgagtgtggggtgggctggggcttctggagccctggagcctggcagcaggggctgctcactgctgtgggaccctctgggcttcagtctccctcgtgtccatggggcgtcccccagggtccctgctggccccacatccgacagtctggggccaggtgactcggccgagggaggagtccctgcaccacgctagtttgggtggatgcagggctggctctggagactcagcctttgtctgccggtgcctttcagggtgacacttgagctttgagcttcggttctcctgtgtgaggtcagctcgggattccctcccttcctctcaggagtcagggtgttgcgtttaggcgctgtgggaagctcagggtcagggtctggaacctgtcagtgcccctgctccccaccgctgttccttctgccctcaccttccatgtctcctgctgggggcagcctccctgcacagcgtctcctcagagtccctggagcaaggtaagccttgtctccctacagagccaccatctgcttccaagagtggagccatcgtgcgtctttccggggcctgttctgtggctgctaagggcctggtctccccatcttcacgtcacagcccatcaggacccggcgctgtgtcgggtctcctaccctgcagccgacgcgtgtgaagcctcttccggtcacggtgttcccggggaggagacagacgtgtgtgtttgtgtgtgtgcatgcgtgcttgcatatgtgtgcatgcttgcacgcatgtatgtgtgtgtgtatgctgcctgaggcacacacatctgtctaaagttcgagatgttgaagtgactccctcccctcagaggctgccagttttgagtgtggctagtccccctgccccccacctctgcagagggaagaacaggctgtttctgaggggtcttccatcttccaggtggggacttgcggagctctgacttctctgtggtgtggtagagctcgcccttctgtggaaagagaacagcacaggtacaggggtacagttagattaaggagccgtggcaagggcccacattcagatcaaaccaggaaggaccttacatcacttagaaacgtgggcagaatccctaaagaggcgcttctttggagaggccaagacgtcattaagatgggaaatgccttaatcctcccctggcttggcacaaaataccagagacacatggcaccaagggcaggtgaggacgtgagaccacacttggtgagcgtgcgcggctgaggctgtgtctgcccgaggagtgccccacgcaggggcccatggtgggcgctgggagacacggcagaacagcgccgcttcgtgcacgaacgcctgaagttggaaacagtccccatgtttgtcagcagcagagtggaccagtgaattgtagtgcctggaacccgtaggacacgggacacgggaaaatgacgcacaccccaggagcagcacagggagcccgtttctcaggagcacccgatcagtcacagagtgaggaagagagccaaggcagtgagcagagggaaagccaggggcttgcttatgttgccagaccggctgccagcccctgcccagtccttgtcccagcctcaggacacctcccatctgtacccaaagatttgctgtttggggacagcgtcgcgtggaagccccagatgtggccggggtcagctggcagtgtcagagctgtgttcatcttgtggtcccccagcgagtcaaggtggctgagcaggatggggcgtgggtctgtgagcgatgccagaagacacaggatggaggagcccagagagaacggagggggcaggtcagatgcactcacacgctcaggcttggcaaagccaggcaggcccagagcgattctgtaagggttagggttcagatgagggtgttgagggttagggttagggtggttagggggttaggaatagggtgtttaggtgaggtttaagttggttagagttaggggttaggggtaggagtaggggtacatgtgaaatgggcatgttcacgttatgcttcctgcctagattctctgctcttccttcacttcccaacctgacggagtgcggaccgtgcgcaccgccatacagctcttgccaggctgccctgtgcagcagggcggaggcaggaacgtgtgctctcacttctgccggaatccttgggagggctgcaggataccccaacacctcagttccatcctcagggccacagaagccctcaggggtgtagtcaatggtgactttattcttatttttctgggaggagtaacgcctgtgtggggcaggcctgctccttcagcccgcgtggcttactccttcgccagcagccaaggtactccctctgctaccgtttgagacgtgtggagacatggtttgcgtgccgggcgtgtgtgaagtggaaccactcctgggtgattgggtggacagaatttctgcaaagaggaactacagaggggtaaccgaaagtattaagacgtacaattcgaggggaaataaccaattttatgatactttctgttacggttactattcctgctttccctctgtcgtgtgctgtgtatgaaagaagacgtgtgtagatttcctgatctcttcgccacaattcacactagatccagcttcctacaataactcttagaactttaatgaagtgaatctacaactaaactccctttctggaatcttacttaaggaagcagggcaaggtttttttgtggataaacaaaaataagatgaatgatttttgaactatagtagtcaagaagtgttggtagcaatatcattgaccctgggacgtcacgcgctgaaaaactcgcatcctggtgtctcacaaactggggaagaattggggagttgggcagacggctgcctggaagaattaagcagttggagagatggctgcctggaagaactagggagtcggggagacggctgcttggaagaattggggagttggggagatggctgcctggaagaattggggagtcggggagatggctgcttggaagaattggggagttggggagatggctgcctggaagaattggggagtcggggagatggctgcctggaagaattggggagttggggagacggctgcctggaagaactggggagttgggcagatgactaccttgactttttacaagtagctcctttttctgccccgagtggctcaagttcttgtgttctgtgtgtgatgaggtgaaggctttgggaatctctcaggggcggcaggaggctcaggaggtgccgaatcttcccaggtgaaggcaacatagaatatagatgagcaggtgtctcaggaacagtcagcgacgcagctcctgggaagcagccacagagactggcgggagcctggggatgaggacggaggccttggcgctcagtggagggtctcaggcagcagaggctggcgggaacctggggatgaggaggggactcgctgggtagggggttggggcaggccatggtgcacagtgaagtgtctcaggtagcaggcgagggtctgcgctggaggcatgtgcctgccctgtgtggggcccaccaggaacaaacagctgaccaggcagcagggtgtccctggggccctccacagggccacccagcagggtgggatgaggggtattgaatgcaggccagtccctgcaacagacccacagaaatgagccagtttgcacccaaagccactgagaaattgaaatagtgattttaggcccctcctgcctttggggaggatagttggatggtgtaattcccgggcagaggcagcccagtgccaccctcacctgtgtgtggggtccgcccctttcctgggagctcagcgtggagccaaggggggctggaaagtatcggccaggaagagggtctcctggttcaagcacggacaccccaccctgcagagctgggctgcaggggtaggagggttgggctgacggcgccagccgctgggcagggttctgtgggcttgtgtgatcacttcctcatcggatgccagggtttccgcgcaggcatggagatgggaagcccaggaccatcagagacgcggcccttacaccagctccggctccagagggactgggagggaggtcaggcctgcggctttaaaggttcacacctgaaaaccaaacactgacagaaacagctcagaaaactgttctctaatcccacggcttaggagcctgtcccgcgggtctgagctccccgcaggagccacccagagccgcgtcctcacgaggccgactctgacctgcttgcagcacgtgatgaataatgccagtgacctcgtggctgaattcccaggagactgggaccagagcgtgacgtccccacgtcgatggctgcaaggtgccactccccccaccctacccccactgtccctggggccgggcatactcagaattccagcgcgttcaggctgtggggaggaagtgtgccacagaaccccggggcgctcagggcagctcccacagccacatcgcccgtcttcagaaggggtggggtcctcatggacatgaagctctcacaccccttcaggtcagggatcgctgcccagtgaatttgccgcaaacttggggggaacatcttcctgttttcagagctttgtgggctttagaattggaggtaggggattgcaggcctatactttaatcctagaaaatcggggagaggcgaacagatggtggggaggaatgggggcttttctcacggccacattttaaagtagatgttttacaaaatcccaatgggtggaaggtctccagccaggctgacgaggaacaattgcccctgactatagacccgcctcactaagacccgcctcactacggacccgcttcactacggacccgccccactacagacccgccccactaagacccgccccactacgggcccgcctaagacccgcctcattacggacccgccccactaa

SEQ ID NO: 14345 - RNA, 2798 nt, Homo sapiens
  source 1..2798: mol_type = other RNA
gctgggattacaggcatgagccaccgcgcccggcctactagtgttttatctttgattctctgtcagccctcacccctggttcttgcctttcttgatcaacaccttttcttgcctctgtccccttctctccctgtatctctcactcccctccaacctgggggacagtggtgtggaggaggaaccataggcctgagagtccatctgcactccttcctggagcccagaggcaggagaagggggtggtgtctccagccccctggcactgaggaaaaatggggctcttctcactccacccttcccttcctaccctgcaccaggactgggccacttctgggtggggcggtgggtcacagattggctcacactgagaatgtaagaactgcaaacaaaatttctattaagttttctgtctcaaaaaaaaaaagcgggagggtgaagaaaagagccccatctgcctgggcagtaaatacgaggctgaaagataggacttcatcaggaaccggctcatacaaagtctctcacatacatgttttgtctttccgcctcaacacacactgtccctgtccgagctgtgaatgaaagtgagaatggctgcatagtccgtttagatcccagagcccacaggcggccaggaagagctacgcgcagggtgcttactcagccccaggggaaggacctggaagagtgctgtcccgactcctggtgaccatgttccttcccacctctgtcctgtctcttccctgcatcgcagggagaatcacagtaacccattagacccaggtttcccttctttcatcccctagggcgggggaccccaaaccccaggtactggtccgtggcctgtcaggaacagggccgcatgcaggaagtgagcagcgatggcgctctgatcctgtcacatcagtgggacatttggttctcacagaagcagaagccctcctgtgaactgtgcacaccaggagtgtaggttttgtgtgctccttaggagagtttgactaatgcctgatgatgggagatggaacacttccatcccgaaaccagccccgccctccctctccatggaaaaatggtcttccaggaaaatactccctgttgccaaaaaggttggggatcgctgcactaggagcagttttgctgttttgtagcagcttttcctgaccaggcctggcaaagtctccaaccccacccaccagtgaggccagcttcccacacccactcctgcatacatttctgccctcaccagtgacagatgtctctaaccattagtgccggcaacacataacccaggtagaaccgtgctctgtactggcctgaaacctggcagcttgacacttctgttgccagtcccaggccacacacagccctccctcattctggctttaacagtttctccccattttctgctaggaagacagtaggaaactcccttgcccctacacacacacctgtgtggcttttctttttttggagacagagtcccgctctgtcacccaggctggagtgcagtggcatgatctcggctcactgcaacctccgcctcccgggttcaagcgattctcctgcctcagcctcccgagtagctgggactacaggcatgtgccaccaggcaggactaatttttgtatttttagtagagacgggattttgccatgttggccaggatggtcttgaactcctgacctcaggtgatccacctgcctcggcctcccaaagtgctgggattacaggcgtgagccatcgcgcccagcctgtgtgtggcttttcacctggctctgaggctctaacaaggggccctaggtgagtcagctctcacttgaaccttgctgctgggggctggaagcagcagtcctgaactcaacccacctgtgggtaggatatagttctgggccagggagtgacatgggtcaaaagcttcttcttctcacctagtccagttcttcacaggcctacagacccctgcaaggtttccccagggtctaactttaacccacattgcttcaatctaaacccatttcctttctgtgactacctggatgcacggtttggtacctatttttcttgtctctgtccactttactgtggctgtcttcaaacctttgaccacctccaagccactccgtattctggctggggaccactgccttcttcctgcagcttcctgctctcagcaaacaaccaaagctcccagtctacacagccccactggtctctccaggaccagctcttgattctgcctgtctctgagtgacagcctcctgaccatgtttgtgtttgttcttagagacggaggtcgcactctgtggcccaggctgtcctcgaactccctgggctcaagcgctcttactgccttggcctcccgagtagcgtagctgggactcaggtgcaagccaccgtgcctcacttttatttccaaaaagcatcctgttccctcctgctggagaaactgggctgcccctgggctcttggcctccactttgctccgtgccacccagacttatcctgcaggtctcagctcaaaggtcctttcctcaggaacagctatcctccctccccagaacagatcccgccgcccggtccctattatgcccatacggccgccttctgtagaatgacttgttcgtcatctgccacaagacccaggcttttttacttgctcgccaccattcgcccagaagcagagacttcgctaaaagcacctcaatgaataaatgaataaatggtttgtagacaggcctttgaggttcctgcttctgtgaccagcaccagaatgggtgtcccttctgcacagcctgagtgag

SEQ ID NO: 14346 - RNA, 2009 nt, Homo sapiens
  source 1..2009: mol_type = other RNA
gctgggattacaggcatgagccaccgcgcccggcctccacaaaccttttaagtctacaattttacatagttttccatcagggaggcaagatatatataatttctttttatatttaactaaaggttttaagagggcttagtctgtaaatcagtaacaattagtcataacaccatacaaacacatttaaatattcaggaaagaggtttttaagattattgcttagtcttataaaatggtgaattttaatcaaattgatacctctgtattcttatttatgtttcctatactcttacatcatactgcttggcaagtaatgtaagttttgacataatttaaaaattcaagtagttgtaaacaaatcctaatttgttaacaattcatatattcccctttacttactatactacctcagaattaatcctccttaaaaaagcaatcatcccacatagaaaaaactgcagagcttcatctcttccttaaatattttcaagtaccgtaagaacacaaatccatgaaaaaaactgattaaaattggacatttcattaaaattggacattcacaattagctttactaattatggaataatacaaagacataaaaaaagttccttaatatttctttgcttaacagagaaatacaaagaaatactgcaattatggttatgggctatttttcagcctcttcaagtacaggacacaactatggttcctaccagtagggagaaacgaataatcaatcttacataacacgaaagaaagatgagaggcacaaaaagataaactgactttggcttttaagaacctaatgttaaccctgaaatgccacattcagtaacacaacaacaaaacaaaagatgacagcagcaagccaccacttcacacagtattaaaaattctgaaatacgtaatagccttcctcccatctcccactcaatctgctgtgtcgtctttttgtttttcctgctttttagctgcaggcagttcaaggcttgcccactgcatcggttcagcttttctcatagtgatttcaatctttgttgcagtcatagttaataacttcgctttacatcaatcacaccccataatttcacattttgatcaaattccttctctccttcaaatacaatatgcgcatctaacaatgtgctatttgcttctactcgactaagttctggaagtgaatttttagcctatactgaaatggtaacttcacctccagtctgatgccagtcatgtctacatggaacaacttttttcccagcatcttttttagtccacatgtttctcttttgtacagccctcttggtctaagaatgtattaaaatcagaagtttttcttctacaacagctccagtatttcgtcccctcatggaaaataggtactccagaatgatatacacagacttcttctagactctctagaccccgatatgtctttgaacaccctccattcttacatgaggtcccaatcttaatttcatcattgtcttcttttcttattttcttcattccctgatgacagtttaagtttatcaagtgcttgttttagggaggcagatatttttaattccaaatttgtcattggttcatctgggcttggtctttttatcgcgtctactgtcttaggggcttgaatgtgttcctgaaattttggttttaattcagatagttccttctcctcagtagtcttgacctcaggtttgactggctcaggtggcttctcactattatgtctaccttttgtacagcctacaatgcttaagaaatcagaaaaatcagttgttcttctcttacagcaagaccaaccctttaatgcatcgtgaaagactggaacgcctgggtgatatgtgcaagcatcgtcggaattggtctcaggatcgaagcgctgaccgcagctccggttgtagcacagcaaggccattttttttcccactgtcacaggcaaggcccaaacaccgggaacagcaagaggatgcgttagccaatcccgtgttgctagcaccagtct

SEQ ID NO: 14347 - RNA, 988 nt, Homo sapiens
  source 1..988: mol_type = other RNA
gctgggattacaggcatgagccaccgcgcccggcctccataaatattttaagtgagttgagaagaagtacttagatagttattacccagagattcttcattctgagttaaagtcaccccagatcagcatggcagtaccattctggctgtccagtatcatgtgattctgtgaaagaaatacactcccatcagcagcagtgacctgattgccaggctgtcctcctgaaactggggttcaatcacagagaccgcatagataaaagtcctggagagcttctgagatagctggttgacctgacatgctagatacgggtcaaagatcactcaggaatctgggaatgccttgatgatggactcataggcaggtgggggcggtgttgaaaggcccactcgaagactgttactggaccagtagtcaggacggctcagactgtgggaagtgctgatggtgggagagatattggaagaagggagagtcaccagctgactctcagtttccacaggaagtggtggacattgcagaaagggatggaaagtagaagctctgaaacttgattttcttggaaaggaatttgcttgttccagggaagcttgtcgctggaaggtgagactggccaggctgaggttgcttcgacgttcacagccactgtggcggtaaaatccagttctgttgaggccgtgggtgtaagaagacctagatctcctgcttgaactccactgtgagatgggagcactggctcttcttcttcgagacagacaaatgaacacagcccaaataaatcctccaagtaccagcccgattgccatggatacagtgaaggacatgataaggtcctcccaaaagttttctggccatggactccctaaacttgttgtgttattagccataatatccacaagaaatagaagaaagagaagaaaaacagaaagaaaaaccagtatgtcgaaaaaaagcagtttgattctatctctttgtagtacagcaagag

SEQ ID NO: 14348 - RNA, 4034 nt, Homo sapiens
  source 1..4034: mol_type = other RNA
gctgggattacaggcatgagccaccgcgcccggcctgcagtcagataatttttaacacccaggtcatgacaggcagctcagatcgcatggtaacatggtggcctgttcaagtattcagtttctattaaggcccagtagcaggccaaaagtggtctctcacatggagagcatctgtaaattatggcaggccttgctccaaaaccctaaaggcctgcactgcgattctcctatgggggtctgctaaaggttccaagcagcatccctatctgccactgacatttcaggtaccattgggtctgctggatcctatggctcaggtggcagagaagcttgcacagcaactccctactggggatcctcctcctgttctgggcctcactcaaagctagcagcttttcaggtcactcaggaaaagggccagagtaacatacccaaacgaggcatatgtctcctccaaaatccaaataggcccactaggcattgtgcctctttcttggttgtaggagtggccagatgaaacaacttaccttttgctttagaccttctaaagtaccctacaccactggacccctagaaatttaactaagatgaaaggcccctgaattttagtcagctattcccccatcctctgacatgcaaatgccttatcaatcagtcaagagtagttgctacttgtggctcactagatacaatcagtgtaatgtcatcaatgtaatgaagcagtgtgacatcttgtggaaggaaaaggtgatcaagatgcctgcaaactaaattataacagggctggagggttgatatattcctgagggtaggacgatgaaggtgtattgctggcttgccaattgagagcaaaccatcacacaaaaccaaaagcattgctgatactaccctggtctgccgtccacactcacaaagcaggggaatgctgaatctcagggctttgtgaaaatgaaaatgtaatctctttccgctcaagttcatgaaactctgaattgtgtccaaggatgctttgggatctgtagacaaaagatgcttattcttctcatgtgaaatgtgttctggaaactgtagttcaggatgagtatagatgctcaaggaagaagtgaggacccacacttccaggttcttgtcctgatatctttagagtgtgagttttgccttcacagttgcaaaatggctgtagcacttccagacatttcttcatgtgctaagtgctttttcttcggtggtccatttgtcagcatcttggatgtctccaagctctccagctttctgggattaaatcatccttgaacactcaaactttcacaggaatctggacgctgctcagccggctgttgactgggaggaacgattggtgggctcaacatatttaaccagtcccggggattagaaggagaaggtgggttcatttctttctgatagtggcgaccctggttgacagggggtggcaggcaggagttccaggtggttgtgtcgtcactgctggtacttatgctgacattacagttgtccacctgggaggcactcaggccatgggaggtcccagcatcctccagttcttcattttgttgccaccgtaggcttgctagcatctgtaactcggattcactcatctggcttggctgatagtttcgccagtcatattcagatgcttcggggatcgagctcagcctttcccctgagatttctttcagggaggttttgtttagtgaagctggcacttgctgggctgatagatccttcgctttgattacgggctctggagttttctgacaggacccacaccttcttccagttggagaaaggcatgttgtaggcaacaaactcatttcaaagttatttctatctatttgctccatcgaggaatcctggctttctgttgctcctgcttctgtgtaggcgctccttagatattccttacttgtccgctttgcagccttccccagcaggctctctaatgttaactgagttaactctgaaggaccagttgttgggcctcgagaaccctggatactgtggttaccctcttcactgctgtcgccgccgtaaaaatcatcctctgattgggtgtctctgcttgtcacactgttatcctcttttagatccaaaataaatgagagctcctctggggacatagtctgagtctttccatgaggtgctgatcgtggtcttgatgaaaaagtgaaaatgtcctttggaacactctgggattcctctgcctgctggtcgtgttcactctctttgctggcttccagccacaggtgtgatgggttgcaggagtcatcacccagaagtagagactgtctgctggatgccagatatgaaatgtgatcagcattttcaggaaaaatccactcatctgattgatcaggagactggggtcctagagtgccggagttcaacagctctgctccttgttgggacacagtggtgaggatagttgatgctttatcttcaatcctattatttcctgaagagctaccgctgggtgtctctgtcctttctctgctggtactttttaaccgtaatcttcttctgttattattcttatctgctgatggttcttgagggggatgcggatgcataatatgtagattggctgcatgaataggtacagtctgctttatttggtgaatattttctttatttccttgttcctcagactcaggtatcagcaaggctgacatttctgtaccattaacacacttctctacagtggacggctggcatgatcggttatttttggacccaacggatctcactgtctcgctggatatcttcatgttattccttctgccagagagtggaggtggcccaagaactttggatccaaatgcgatatgacaaacatcttgatttttactgttccgtgtaatacttgttcctctgttaatgaactgatctgattctgctgatcttagaggatggcctccgaattttatttcagtttggcgaagtttagtcatgtttagcagctgtgtgacatgtggaacatctgtcattagttgacagcttcgtggtataatatctgtaggctcatctgttgaaaagggaacaccatagacagcatccttatcagcagtgtcttgtggctttgattttaaggtgaagatcttccgtagcttacagttagctgagacaacaattccatccaatgactggaaaactgcccccttgaatatttcactggtgaatgctactaagtcaatgcatagattgcaccaaattttacgtttgatcatgaagagtggaatttttgcatgaagaggggtggaggatagttccttatggaccgttgataaatataatcttcttttgatgttccctaaatcagtaattagcaattcagtggagaagtcttgtcccaggggtacgtaaatctgaagtacaagaaacctctggatcaatccaaggctttgcttattctcctttggtaactgaattttgtttgtttggctgctgccttccaggacaaacacaaaacttttaacttctttatcaaactctttccaaatcacagatggactaccaaggatcttccattttgctccaggattttttccttgagcactgaaaatttcaacaaatgcacctccctggtactcatttttgaacattcccgcagggggcccagggcttggggggcacagagttcagggtttccagcgagtggcgtgaccctgacggctggaaatcggctggcgggaacccaggagcccgacgggtgggaaagggcttcgtgcttggcccagacttgggcaggctcttctcagcccctccggcccctggtcagctccatctcccgccctccatcagcaccattgcggctccagcctccgcggtgcccgggtctggggagggcgcagctgcctggacggactccgggccgtccctggggagtgattgtgtgtgtaacctacgtgacggggcgcccagtcgcggagccacagacaaccgcccgctggcctaggaaaagcgggcgcgctcccgctgccgccccaccccagaatcaaaccgcgaaagagcagcgc

SEQ ID NO: 14349 - RNA, 3972 nt, Homo sapiens
  source 1..3972: mol_type = other RNA
gctgggattacaggcatgagccaccgcgcccggcctgcagtcagataatttttaacacccaggtcatgacaggcagctcagatcgcatggtaacatggtggcctgttcaagtattcagtttctattaaggcccagtagcaggccaaaagtggtctctcacatggagagcatctgtaaattatggcaggccttgctccaaaaccctaaaggcctgcactgcgattctcctatgggggtctgctaaaggttccaagcagcatccctatctgccactgacatttcaggtaccattgggtctgctggatcctatggctcaggtggcagagaagcttgcacagcaactccctactggggatcctcctcctgttctgggcctcactcaaagctagcagcttttcaggtcactcaggaaaagggccagagtaacatacccaaacgaggcatatgtctcctccaaaatccaaataggcccactaggcattgtgcctctttcttggttgtaggagtggccagatgaaacaacttaccttttgctttagaccttctaaagtaccctacaccactggacccctagaaatttaactaagatgaaaggcccctgaattttagtcagctattcccccatcctctgacatgcaaatgccttatcaatcagtcaagagtagttgctacttgtggctcactagatacaatcagtgtaatgtcatcaatgtaatgaagcagtgtgacatcttgtggaaggaaaaggtgatcaagatgcctgcaaactaaattataacagggctggagggttgatatattcctgagggtaggacgatgaaggtgtattgctggcttgccaattgagagcaaaccatcacacaaaaccaaaagcattgctgatactaccctggtctgccgtccacactcacaaagcaggggaatgctgaatctcagggctttgtgaaaatgaaaatgtaatctctttccgctcaagttcatgaaactctgaattgtgtccaaggatgctttgggatctgtagacaaaagatgcttattcttctcatgtgaaatgtgttctggaaactgtagttcaggatgagtatagatgctcaaggaagaagtgaggacccacacttccaggttcttgtcctgatatctttagagtgtgagttttgccttcacagttgcaaaatggctgtagcacttccagacatttcttcatgtgctaagtgctttttcttcggtggtccatttgtcagcatcttggatgtctccaagctctccagctttctgggattaaatcatccttgaacactcaaactttcacaggaatctggacgctgctcagccggctgttgactgggaggaacgattggtgggctcaacatatttaaccagtccgggtggcaggcaggagttccaggtggttgtgtcgtcactgctggtacttatgctgacattacagttgtccacctgggaggcactcaggccatgggaggtcccagcatcctccagttcttcattttgttgccaccgtaggcttgctagcatctgtaactcggattcactcatctggcttggctgatagtttcgccagtcatattcagatgcttcggggatcgagctcagcctttcccctgagatttctttcagggaggttttgtttagtgaagctggcacttgctgggctgatagatccttcgctttgattacgggctctggagttttctgacaggacccacaccttcttccagttggagaaaggcatgttgtaggcaacaaactcatttcaaagttatttctatctatttgctccatcgaggaatcctggctttctgttgctcctgcttctgtgtaggcgctccttagatattccttacttgtccgctttgcagccttccccagcaggctctctaatgttaactgagttaactctgaaggaccagttgttgggcctcgagaaccctggatactgtggttaccctcttcactgctgtcgccgccgtaaaaatcatcctctgattgggtgtctctgcttgtcacactgttatcctcttttagatccaaaataaatgagagctcctctggggacatagtctgagtctttccatgaggtgctgatcgtggtcttgatgaaaaagtgaaaatgtcctttggaacactctgggattcctctgcctgctggtcgtgttcactctctttgctggcttccagccacaggtgtgatgggttgcaggagtcatcacccagaagtagagactgtctgctggatgccagatatgaaatgtgatcagcattttcaggaaaaatccactcatctgattgatcaggagactggggtcctagagtgccggagttcaacagctctgctccttgttgggacacagtggtgaggatagttgatgctttatcttcaatcctattatttcctgaagagctaccgctgggtgtctctgtcctttctctgctggtactttttaaccgtaatcttcttctgttattattcttatctgctgatggttcttgagggggatgcggatgcataatatgtagattggctgcatgaataggtacagtctgctttatttggtgaatattttctttatttccttgttcctcagactcaggtatcagcaaggctgacatttctgtaccattaacacacttctctacagtggacggctggcatgatcggttatttttggacccaacggatctcactgtctcgctggatatcttcatgttattccttctgccagagagtggaggtggcccaagaactttggatccaaatgcgatatgacaaacatcttgatttttactgttccgtgtaatacttgttcctctgttaatgaactgatctgattctgctgatcttagaggatggcctccgaattttatttcagtttggcgaagtttagtcatgtttagcagctgtgtgacatgtggaacatctgtcattagttgacagcttcgtggtataatatctgtaggctcatctgttgaaaagggaacaccatagacagcatccttatcagcagtgtcttgtggctttgattttaaggtgaagatcttccgtagcttacagttagctgagacaacaattccatccaatgactggaaaactgcccccttgaatatttcactggtgaatgctactaagtcaatgcatagattgcaccaaattttacgtttgatcatgaagagtggaatttttgcatgaagaggggtggaggatagttccttatggaccgttgataaatataatcttcttttgatgttccctaaatcagtaattagcaattcagtggagaagtcttgtcccaggggtacgtaaatctgaagtacaagaaacctctggatcaatccaaggctttgcttattctcctttggtaactgaattttgtttgtttggctgctgccttccaggacaaacacaaaacttttaacttctttatcaaactctttccaaatcacagatggactaccaaggatcttccattttgctccaggattttttccttgagcactgaaaatttcaacaaatgcacctccctggtactcatttttgaacattcccgcagggggcccagggcttggggggcacagagttcagggtttccagcgagtggcgtgaccctgacggctggaaatcggctggcgggaacccaggagcccgacgggtgggaaagggcttcgtgcttggcccagacttgggcaggctcttctcagcccctccggcccctggtcagctccatctcccgccctccatcagcaccattgcggctccagcctccgcggtgcccgggtctggggagggcgcagctgcctggacggactccgggccgtccctggggagtgattgtgtgtgtaacctacgtgacggggcgcccagtcgcggagccacagacaaccgcccgctggcctaggaaaagcgggcgcgctcccgctgccgccccaccccagaatcaaaccgcgaaagagcagcgc

SEQ ID NO: 14350 - RNA, 3267 nt, Homo sapiens
  source 1..3267: mol_type = other RNA
gctgggattacaggcatgagccaccgcgcccggcctgctctaacttattttaagaatcactgttctattctggaaagggaaaagaccaccaccaagaagggaaaggagaccatgctggacagcctaatagtctaacaggggatcctagggtgcctgagctcatgggagcaaaccttgttcaggcaccgcaagcccaacgcagcatgcagattgggaaggcgcaataatgcaaacaccatcaggaagaaagctatggatgatggaaaacactgtgtgctccacgtgacagaagggagccacctgatttgtcgcatcgggccagtgtaaggaagtgtaatttagtgggactgccagtgacactaagtcaggccttgatcagggtctggactcagtatggacacgagccactgggtgcagggggctcatgcctgccacctctctttttttcccttactatagagactttgatctgtccaccatttctatgtgagctttgggcttcctgtcacaggtctgttgtcaccgtggggccatgttggagtcggtagattttcagacagtgaagccacatgaagctgtgaatgctgatgtggctgctgcagagcccagtctctccccggtgcagggcctctgagacgacgggactgtcctcagatggttggaagaaatgggttatcttaggcagttaggaaaagagggacaggtgtcccaggatgtggaaaacttgagttcatcccctctcttccctccagcaaggatttcagtgctacatctaaaaagagaagccctgttgccgatttaataatttacagtctctaaatccaaaagggcctccatgtgctagtgagactcatgccctcagttatgttcacgatcttcctgagaagtcagacaatacaggtagaacaaaagatagtggttgtactttctcttctgcgtagtgtgggtaagagcatgcggtttgccgcatgcagtgttgttaatcttttgattgtgttgtgaatggctgaaaaaaaagctgaaagtttgattgaactgaaatccaatccatgtcaacataaggaatattctagtgagtttactgtcctaagagaaggtctctcctggggaacccctggtatgcagagctccctgggacttgcagattggacagagagggtgtgccaaaggggtataaacccttctgatggagagagtcgggcgtgtcttcattttggtagttctggaaaggctcctctttaaagattctgatttaataatgttcacttttgttaagattgaatatcattttgaaatcatttctaaacgtgtttcctttataggcactttatctattaaatttacagtggagccaaatgtattagcaaaatctccaagttgcaaaatgaatactcagaatcaaactatagattttttggtgatactttcagaaaaacaatttctttctaaagttgcaaatcatgaaagggaatgaaagtacattaacttgatttcttccctgtaattcaaacattcaacattcaaattaactttcataatttctcactttgtgacaagttgatttacgcatagttggtatttcattaatgcgatttatatagatggaattcttaaggataaacaaatgtttttgactattgcctggggttctttgggaatagatgctttctgaaaatttaaataagaacattactgttaaagccatgaatctagtttggagaacccactgcagttcattttacagagaaacaccttgtcaatggcatcttcatggtgtttactgaaggtaaaaggcaggatattaaatgtgagaactctctctccagctactgattctgcctgtctcgaattcaggtgagaatgacccatacagatacatggattgcacttgaatctgtgctctggtatttgtgtcatccggaggctgagaacgcctgttggtggtgtcgcagatggctctgctgtcttgtgtggacaaactgaaagggattcaggagcttcttctgtaattttactctgctgtttttcatggacatagtgaaagggatccaggagtttcttctgcaatttggctgtagttggactttgaaaaaaacttgaagagtgtgtgtgcgcgcgcgcgcgtgtgtgtgtgtgtttgaaaagagaattagaaaatgaaggtagacactgggtatgctcccccaggatgtggcgatggggcgcccggccgccctggctacacgtcgaaccagtggtcccccatgcagacgcggttccactcgcagccacagttccagcaccactcgagcctgcactggggctgcggacacttcatgtgcatgcagcctccatttttttccactggtacatggcagcggggacagggcttggtggttttcttgatggtttctttggaggctgcttcccaacgagcctgctcggcggctctttcatcgactctgtaggcctgagtagttgttcctgaggcttcaaatacggcactgcactccccttcatggtacgcttctttacattcccggcagaaggcaaacccacagcccaggccattgcccccttcgcaggtgactttcctctggtcaggctccggcagcagccccgctccacagccagggcgggggcataacacgccccccatctgcaggacacactcctctgcaccatactgctggtaccggttgtactgctcttctcccagaatcctgaagtgatggagctctttaatcaaggagttgggacagccagccacacaaggcagggagtagccaagttgagggtcgtgaacaaactgccgatcattgagtcttgtcacacagtataagtggaaacagtctaagcaaatcacgtggcgggagttgcactggaaaaccaggacggggctcctgacgtctgtgcacgtaatgcaagtgatgttccgactatttgttgcgatcaggtgcaaagctactgatgtttccttgtcagaggtggggtgtgctccacatttaaagaaaaattcctgcacagtccagtcattcctcagctccttccctgcgaaaatcacacgcaactggtcagccggaaccccctgtcgcttagcaaccacctccttgagctggaagatgctggtgtcagaatcgacctccactgggaaaccatggctggagttgaacctgacaaacactatcatggtcactgggtaggtggcggctgcgggccaggaacaggcccatgcgcgcagcggcgccagccgcgcctcccaccagcggctctcctgggttaaatcct

SEQ ID NO: 14351 - RNA, 3630 nt, Homo sapiens
  source 1..3630: mol_type = other RNA
gctgggattacaggcatgagccaccgcgcccggcctgctctaacttattttaagaatcactgttctattctggaaagggaaaagaccaccaccaagaagggaaaggagaccatgctggacagcctaatagtctaacaggggatcctagggtgcctgagctcatgggagcaaaccttgttcaggcaccgcaagcccaacgcagcatgcagattgggaaggcgcaataatgcaaacaccatcaggaagaaagctatggatgatggaaaacactgtgtgctccacgtgacagaagggagccacctgatttgtcgcatcgggccagtgtaaggaagtgtaatttagtgggactgccagtgacactaagtcaggccttgatcagggtctggactcagtatggacacgagccactgggtgcagggggctcatgcctgccacctctctttttttcccttactatagagactttgatctgtccaccatttctatgtgagctttgggcttcctgtcacaggtctgttgtcaccgtggggccatgttggagtcggtagattttcagacagtgaagccacatgaagctgtgaatgctgatgtggctgctgcagagcccagtctctccccggtgcagggcctctgagacgacgggactgtcctcagatggttggaagaaatgggttatcttaggcagttaggaaaagagggacaggtgtcccaggatgtggaaaacttgagttcatcccctctcttccctccagcaaggatttcagtgctacatctaaaaagagaagccctgttgccgatttaataatttacagtctctaaatccaaaagggcctccatgtgctagtgagactcatgccctcagttatgttcacgatcttcctgagaagtcagacaatacaggtagaacaaaagatagtggttgtactttctcttctgcgtagtgtgggtaagagcatgcggtttgccgcatgcagtgttgttaatcttttgattgtgttgtgaatggctgaaaaaaaagctgaaagtttgattgaactgaaatccaatccatgtcaacataaggaatattctagtgagtttactgtcctaagagaaggtctctcctggggaacccctggtatgcagagctccctgggacttgcagattggacagagagggtgtgccaaaggggtataaacccttctgatggagagagtcgggcgtgtcttcattttggtagttctggaaaggctcctctttaaagattctgatttaataatgttcacttttgttaagattgaatatcattttgaaatcatttctaaacgtgtttcctttataggcactttatctattaaatttacagtggagccaaatgtattagcaaaatctccaagttgcaaaatgaatactcagaatcaaactatagattttttggtgatactttcagaaaaacaatttctttctaaagttgcaaatcatgaaagggaatgaaagtacattaacttgatttcttccctgtaattcaaacattcaacattcaaattaactttcataatttctcactttgtgacaagttgatttacgcatagttggtatttcattaatgcgatttatatagatggaattcttaaggataaacaaatgtttttgactattgcctggggttctttgggaatagatgctttctgaaaatttaaataagaacattactgttaaagccatgaatctagtttggagaacccactgcagttcattttacagagaaacaccttgtcaatggcatcttcatggtgtttactgaaggtaaaaggcaggatattaaatgtgagaactctctctccagctactgattctgcctgtctcgaattcaggtgagaatgacccatacagatacatggattgcacttgaatctgtgctctggtatttgtgtcatccggaggctgagaacgcctgttggtggtgtcgcagatggctctgctgtcttgtgtggacaaactgaaagggattcaggagcttcttctgtaattttactctgctgtttttcatggacatagtgaaagggatccaggagtttcttctgcaatttggctgtagttggactttgaaaaaaacttgaagagtgtgtgtgcgcgcgcgcgcgtgtgtgtgtgtgtttgaaaagagaattagaaaatgaaggtagacactgggtatgctcccccaggatgtggcgatggggcgcccggccgccctggctacacgtcgaaccagtggtcccccatgcagacgcggttccactcgcagccacagttccagcaccactcgagcctgcactggggctgcggacacttcatgtgcatgcagcctccatttttttccactggtacatggcagcggggacagggcttggtggttttcttgatggtttctttggaggctgcttcccaacgagcctgctcggcggctctttcatcgactctgtaggcctgagtagttgttcctgaggcttcaaatacggcactgcactccccttcatggtacgcttctttacattcccggcagaaggcaaacccacagcccaggccattgcccccttcgcaggtgactttcctctggtcaggctccggcagcagccccgctccacagccagggcgggggcataacacgccccccatctgcaggacacactcctctgcaccatactgctggtaccggttgtactgctcttctcccagaatcctgaagtgatggagctctttaatcaaggagttgggacagccagccacacaaggcagggagtagccaagttgagggtcgtgaacaaactgccgatcattgagtcttgtcacacagtataagtggaaacagtctaagcaaatcacgtggcgggagttgcactggaaaaccaggacggggctcctgacgtctgtgcacgtaatgcaagtgatgttccgactatttgttgcgatcaggtgcaaagctactgatgtttccttgtcagaggtggggtgtgctccacatttaaagaaaaattcctgggtcaaggtgagcgttgcctgcctgcaggtgctgcactgtaccctgagttttcccggctgcactctttgacaggggcctttgcaatacacataaaagctgttgtagattgatctacctgctggacttccagctggtggtgagtccttcctgctgtcagtgtgcagaatgacagccagccccacagagtctcctgggaggactgagctgctgaggtccacccgagtcaagctctggggctcccgctcacagcctcccgccgcgtttctggggtcgtcgcctccagttgcattcatttcttgaccttttctccacggtctctgcacaatgtgaacaatgctctgctgatccaggtcacaattctgcacagtccagtcattcctcagctccttccctgcgaaaatcacacgcaactggtcagccggaaccccctgtcgcttagcaaccacctccttgagctggaagatgctggtgtcagaatcgacctccactgggaaaccatggctggagttgaacctgacaaacactatcatggtcactgggtaggtggcggctgcgggccaggaacaggcccatgcgcgcagcggcgccagccgcgcctcccaccagcggctctcctgggttaaatcct

SEQ ID NO: 14352 - RNA, 3562 nt, Homo sapiens
  source 1..3562: mol_type = other RNA
gctgggattacaggcatgagccaccgcgcccggcctgctctaacttattttaagaatcactgttctattctggaaagggaaaagaccaccaccaagaagggaaaggagaccatgctggacagcctaatagtctaacaggggatcctagggtgcctgagctcatgggagcaaaccttgttcaggcaccgcaagcccaacgcagcatgcagattgggaaggcgcaataatgcaaacaccatcaggaagaaagctatggatgatggaaaacactgtgtgctccacgtgacagaagggagccacctgatttgtcgcatcgggccagtgtaaggaagtgtaatttagtgggactgccagtgacactaagtcaggccttgatcagggtctggactcagtatggacacgagccactgggtgcagggggctcatgcctgccacctctctttttttcccttactatagagactttgatctgtccaccatttctatgtgagctttgggcttcctgtcacaggtctgttgtcaccgtggggccatgttggagtcggtagattttcagacagtgaagccacatgaagctgtgaatgctgatgtggctgctgcagagcccagtctctccccggtgcagggcctctgagacgacgggactgtcctcagatggttggaagaaatgggttatcttaggcagttaggaaaagagggacaggtgtcccaggatgtggaaaacttgagttcatcccctctcttccctccagcaaggatttcagtgctacatctaaaaagagaagccctgttgccgatttaataatttacagtctctaaatccaaaagggcctccatgtgctagtgagactcatgccctcagttatgttcacgatcttcctgagaagtcagacaatacaggtagaacaaaagatagtggttgtactttctcttctgcgtagtgtgggtaagagcatgcggtttgccgcatgcagtgttgttaatcttttgattgtgttgtgaatggctgaaaaaaaagctgaaagtttgattgaactgaaatccaatccatgtcaacataaggaatattctagtgagtttactgtcctaagagaaggtctctcctggggaacccctggtatgcagagctccctgggacttgcagattggacagagagggtgtgccaaaggggtataaacccttctgatggagagagtcgggcgtgtcttcattttggtagttctggaaaggctcctctttaaagattctgatttaataatgttcacttttgttaagattgaatatcattttgaaatcatttctaaacgtgtttcctttataggcactttatctattaaatttacagtggagccaaatgtattagcaaaatctccaagttgcaaaatgaatactcagaatcaaactatagattttttggtgatactttcagaaaaacaatttctttctaaagttgcaaatcatgaaagggaatgaaagtacattaacttgatttcttccctgtaattcaaacattcaacattcaaattaactttcataatttctcactttgtgacaagttgatttacgcatagttggtatttcattaatgcgatttatatagatggaattcttaaggataaacaaatgtttttgactattgcctggggttctttgggaatagatgctttctgaaaatttaaataagaacattactgttaaagccatgaatctagtttggagaacccactgcagttcattttacagagaaacaccttgtcaatggcatcttcatggtgtttactgaaggtaaaaggcaggatattaaatgtgagaactctctctccagctactgattctgcctgtctcgaattcaggtgagaatgacccatacagatacatggattgcacttgaatctgtgctctggtatttgtgtcatccggaggctgagaacgcctgttggtggtgtcgcagatggctctgctgtcttgtgtggacaaactgaaagggattcaggagcttcttctgtaattttactctgctgtttttcatggacatagtgaaagggatccaggagtttcttctgcaatttggctgtagttggactttgaaaaaaacttgaagagtgtgtgtgcgcgcgcgcgcgtgtgtgtgtgtgtttgaaaagagaattagaaaatgaaggtagacactgggtatgctcccccaggatgtggcgatggggcgcccggccgccctggctacacgtcgaaccagtggtcccccatgcagacgcggttccactcgcagccacagttccagcaccactcgagcctgcactggggctgcggacacttcatgtgcatgcagcctccatttttttccactggtacatggcagcggggacagggcttggtggttttcttgatggtttctttggaggctgcttcccaacgagcctgctcggcggctctttcatcgactctgtaggcctgagtagttgttcctgaggcttcaaatacggcactgcactccccttcatggtacgcttctttacattcccggcagaaggcaaacccacagcccaggccattgcccccttcgcaggtgactttcctctggtcaggctccggcagcagccccgctccacagccagggcgggggcataacacgccccccatctgcaggacacactcctctgcaccatactgctggtaccggttgtactgctcttctcccagaatcctgaagtgatggagctctttaatcaaggagttgggacagccagccacacaaggcagggagtagccaagttgagggtcgtgaacaaactgccgatcattgagtcttgtcacacagtataagtggaaacagtctaagcaaatcacgtggcgggagttgcactggaaaaccaggacggggctcctgacgtctgtgcacgtaatgcaagtgatgttccgactatttgttgcgatcaggtgcaaagctactgatgtttccttgtcagaggtggggtgtgctccacatttaaagaaaaattctgcactagtcccagggcagtgtggggattggcattcaccactcatccggtttggaattaaaacatcatcccagcaagatggaccctgggtcaaggtgagcgttgcctgcctgcaggtgctgcactgtaccctgagttttcccggctgcactctttgacaggggcctttgcaatacacataaaagctgttgtagattgatctacctgctggacttccagctggtggtgagtccttcctgctgtcagtgtgcagaatgacagccagccccacagagtctcctgggaggactgagctgctgaggtccacccgagtcaagctctggggctcccgctcacagcctcccgccgcgtttctggggtcgtcgcctccagttgcattcatttcttgaccttttctccacggtctctgcacaatgtgaacaatgctctgctgatccaggtcacaattctatcatggtcactgggtaggtggcggctgcgggccaggaacaggcccatgcgcgcagcggcgccagccgcgcctcccaccagcggctctcctgggttaaatcctccaggcctcccc

SEQ ID NO: 14353 - RNA, 3714 nt, Homo sapiens
  source 1..3714: mol_type = other RNA
gctgggattacaggcatgagccaccgcgcccggcctgctctaacttattttaagaatcactgttctattctggaaagggaaaagaccaccaccaagaagggaaaggagaccatgctggacagcctaatagtctaacaggggatcctagggtgcctgagctcatgggagcaaaccttgttcaggcaccgcaagcccaacgcagcatgcagattgggaaggcgcaataatgcaaacaccatcaggaagaaagctatggatgatggaaaacactgtgtgctccacgtgacagaagggagccacctgatttgtcgcatcgggccagtgtaaggaagtgtaatttagtgggactgccagtgacactaagtcaggccttgatcagggtctggactcagtatggacacgagccactgggtgcagggggctcatgcctgccacctctctttttttcccttactatagagactttgatctgtccaccatttctatgtgagctttgggcttcctgtcacaggtctgttgtcaccgtggggccatgttggagtcggtagattttcagacagtgaagccacatgaagctgtgaatgctgatgtggctgctgcagagcccagtctctccccggtgcagggcctctgagacgacgggactgtcctcagatggttggaagaaatgggttatcttaggcagttaggaaaagagggacaggtgtcccaggatgtggaaaacttgagttcatcccctctcttccctccagcaaggatttcagtgctacatctaaaaagagaagccctgttgccgatttaataatttacagtctctaaatccaaaagggcctccatgtgctagtgagactcatgccctcagttatgttcacgatcttcctgagaagtcagacaatacaggtagaacaaaagatagtggttgtactttctcttctgcgtagtgtgggtaagagcatgcggtttgccgcatgcagtgttgttaatcttttgattgtgttgtgaatggctgaaaaaaaagctgaaagtttgattgaactgaaatccaatccatgtcaacataaggaatattctagtgagtttactgtcctaagagaaggtctctcctggggaacccctggtatgcagagctccctgggacttgcagattggacagagagggtgtgccaaaggggtataaacccttctgatggagagagtcgggcgtgtcttcattttggtagttctggaaaggctcctctttaaagattctgatttaataatgttcacttttgttaagattgaatatcattttgaaatcatttctaaacgtgtttcctttataggcactttatctattaaatttacagtggagccaaatgtattagcaaaatctccaagttgcaaaatgaatactcagaatcaaactatagattttttggtgatactttcagaaaaacaatttctttctaaagttgcaaatcatgaaagggaatgaaagtacattaacttgatttcttccctgtaattcaaacattcaacattcaaattaactttcataatttctcactttgtgacaagttgatttacgcatagttggtatttcattaatgcgatttatatagatggaattcttaaggataaacaaatgtttttgactattgcctggggttctttgggaatagatgctttctgaaaatttaaataagaacattactgttaaagccatgaatctagtttggagaacccactgcagttcattttacagagaaacaccttgtcaatggcatcttcatggtgtttactgaaggtaaaaggcaggatattaaatgtgagaactctctctccagctactgattctgcctgtctcgaattcaggtgagaatgacccatacagatacatggattgcacttgaatctgtgctctggtatttgtgtcatccggaggctgagaacgcctgttggtggtgtcgcagatggctctgctgtcttgtgtggacaaactgaaagggattcaggagcttcttctgtaattttactctgctgtttttcatggacatagtgaaagggatccaggagtttcttctgcaatttggctgtagttggactttgaaaaaaacttgaagagtgtgtgtgcgcgcgcgcgcgtgtgtgtgtgtgtttgaaaagagaattagaaaatgaaggtagacactgggtatgctcccccaggatgtggcgatggggcgcccggccgccctggctacacgtcgaaccagtggtcccccatgcagacgcggttccactcgcagccacagttccagcaccactcgagcctgcactggggctgcggacacttcatgtgcatgcagcctccatttttttccactggtacatggcagcggggacagggcttggtggttttcttgatggtttctttggaggctgcttcccaacgagcctgctcggcggctctttcatcgactctgtaggcctgagtagttgttcctgaggcttcaaatacggcactgcactccccttcatggtacgcttctttacattcccggcagaaggcaaacccacagcccaggccattgcccccttcgcaggtgactttcctctggtcaggctccggcagcagccccgctccacagccagggcgggggcataacacgccccccatctgcaggacacactcctctgcaccatactgctggtaccggttgtactgctcttctcccagaatcctgaagtgatggagctctttaatcaaggagttgggacagccagccacacaaggcagggagtagccaagttgagggtcgtgaacaaactgccgatcattgagtcttgtcacacagtataagtggaaacagtctaagcaaatcacgtggcgggagttgcactggaaaaccaggacggggctcctgacgtctgtgcacgtaatgcaagtgatgttccgactatttgttgcgatcaggtgcaaagctactgatgtttccttgtcagaggtggggtgtgctccacatttaaagaaaaattctgcactagtcccagggcagtgtggggattggcattcaccactcatccggtttggaattaaaacatcatcccagcaagatggaccctgggtcaaggtgagcgttgcctgcctgcaggtgctgcactgtaccctgagttttcccggctgcactctttgacaggggcctttgcaatacacataaaagctgttgtagattgatctacctgctggacttccagctggtggtgagtccttcctgctgtcagtgtgcagaatgacagccagccccacagagtctcctgggaggactgagctgctgaggtccacccgagtcaagctctggggctcccgctcacagcctcccgccgcgtttctggggtcgtcgcctccagttgcattcatttcttgaccttttctccacggtctctgcacaatgtgaacaatgctctgctgatccaggtcacaattctgcacagtccagtcattcctcagctccttccctgcgaaaatcacacgcaactggtcagccggaaccccctgtcgcttagcaaccacctccttgagctggaagatgctggtgtcagaatcgacctccactgggaaaccatggctggagttgaacctgacaaacactatcatggtcactgggtaggtggcggctgcgggccaggaacaggcccatgcgcgcagcggcgccagccgcgcctcccaccagcggctctcctgggttaaatcct

SEQ ID NO: 14354 - RNA, 4664 nt, Homo sapiens
  source 1..4664: mol_type = other RNA
gctgggattacaggcatgagccaccgcgcccggcctgctctaacttattttaagaatcactgttctattctggaaagggaaaagaccaccaccaagaagggaaaggagaccatgctggacagcctaatagtctaacaggggatcctagggtgcctgagctcatgggagcaaaccttgttcaggcaccgcaagcccaacgcagcatgcagattgggaaggcgcaataatgcaaacaccatcaggaagaaagctatggatgatggaaaacactgtgtgctccacgtgacagaagggagccacctgatttgtcgcatcgggccagtgtaaggaagtgtaatttagtgggactgccagtgacactaagtcaggccttgatcagggtctggactcagtatggacacgagccactgggtgcagggggctcatgcctgccacctctctttttttcccttactatagagactttgatctgtccaccatttctatgtgagctttgggcttcctgtcacaggtctgttgtcaccgtggggccatgttggagtcggtagattttcagacagtgaagccacatgaagctgtgaatgctgatgtggctgctgcagagcccagtctctccccggtgcagggcctctgagacgacgggactgtcctcagatggttggaagaaatgggttatcttaggcagttaggaaaagagggacaggtgtcccaggatgtggaaaacttgagttcatcccctctcttccctccagcaaggatttcagtgctacatctaaaaagagaagccctgttgccgatttaataatttacagtctctaaatccaaaagggcctccatgtgctagtgagactcatgccctcagttatgttcacgatcttcctgagaagtcagacaatacaggtagaacaaaagatagtggttgtactttctcttctgcgtagtgtgggtaagagcatgcggtttgccgcatgcagtgttgttaatcttttgattgtgttgtgaatggctgaaaaaaaagctgaaagtttgattgaactgaaatccaatccatgtcaacataaggaatattctagtgagtttactgtcctaagagaaggtctctcctggggaacccctggtatgcagagctccctgggacttgcagattggacagagagggtgtgccaaaggggtataaacccttctgatggagagagtcgggcgtgtcttcattttggtagttctggaaaggctcctctttaaagattctgatttaataatgttcacttttgttaagattgaatatcattttgaaatcatttctaaacgtgtttcctttataggcactttatctattaaatttacagtggagccaaatgtattagcaaaatctccaagttgcaaaatgaatactcagaatcaaactatagattttttggtgatactttcagaaaaacaatttctttctaaagttgcaaatcatgaaagggaatgaaagtacattaacttgatttcttccctgtaattcaaacattcaacattcaaattaactttcataatttctcactttgtgacaagttgatttacgcatagttggtatttcattaatgcgatttatatagatggaattcttaaggataaacaaatgtttttgactattgcctggggttctttgggaatagatgctttctgaaaatttaaataagaacattactgttaaagccatgaatctagtttggagaacccactgcagttcattttacagagaaacaccttgtcaatggcatcttcatggtgtttactgaaggtaaaaggcaggatattaaatgtgagaactctctctccagctactgattctgcctgtctcgaattcaggtgagaatgacccatacagatacatggattgcacttgaatctgtgctctggtatttgtgtcatccggaggctgagaacgcctgttggtggtgtcgcagatggctctgctgtcttgtgtggacaaactgaaagggattcaggagcttcttctgtaattttactctgctgtttttcatggacatagtgaaagggatccaggagtttcttctgcaatttggctgtagttggactttgaaaaaaacttgaagagtgtgtgtgcgcgcgcgcgcgtgtgtgtgtgtgtttgaaaagagaattagaaaatgaaggtagacactgggtatgctcccccaggatgtggcgatggggcgcccggccgccctggctacacgtcgaaccagtggtcccccatgcagacgcggttccactcgcagccacagttccagcaccactcgagcctgcactggggctgcggacacttcatgtgcatgcagcctccatttttttccactggtacatggcagcggggacagggcttggtggttttcttgatggtttctttggaggctgcttcccaacgagcctgctcggcggctctttcatcgactctgtaggcctgagtagttgttcctgaggcttcaaatacggcactgcactccccttcatggtacgcttctttacattcccggcagaaggcaaacccacagcccaggccattgcccccttcgcaggtgactttcctctggtcaggctccggcagcagccccgctccacagccagggcgggggcataacacgccccccatctgcaggacacactcctctgcaccatactgctggtaccggttgtactgctcttctcccagaatcctgaagtgatggagctctttaatcaaggagttgggacagccagccacacaaggcagggagtagccaagttgagggtcgtgaacaaactgccgatcattgagtcttgtcacacagtataagtggaaacagtctaagcaaatcacgtggcgggagttgcactggaaaaccaggacggggctcctgacgtctgtgcacgtaatgcaagtgatgttccgactatttgttgcgatcaggtgcaaagctactgatgtttccttgtcagaggtggggtgtgctccacatttaaagaaaaattctgcactagtcccagggcagtgtggggattggcattcaccactcatccggtttggaattaaaacatcatcccagcaagatggaccctgggtcaaggtgagcgttgcctgcctgcaggtgctgcactgtaccctgagttttcccggctgcactctttgacaggggcctttgcaatacacataaaagctgttgtagattgatctacctgctggacttccagctggtggtgagtccttcctgctgtcagtgtgcagaatgacagccagccccacagagtctcctgggaggactgagctgctgaggtccacccgagtcaagctctggggctcccgctcacagcctcccgccgcgtttctggggtcgtcgcctccagttgcattcatttcttgaccttttctccacggtctctgcacaatgtgaacaatgctctgctgatccaggtcacaattctgcacagtccagtcattcctcagctccttccctgcgaaaatcacacgcaactggtcagccggaaccccctgtcgcttagcaaccacctccttgagctggaagatgctggtgtcagaatcgacctccactgggaaaccatggctggagttgaacctgacaaacactgtaattggatattctctttctggcctagtatataacctccctgattcaggctgcggctcagagttcttcaaagagtaagtacagttatcactgttgaaagtgactctggctgtaaacatcaaagacgtgatttctaatgttgttgtggctgaaactccgcttaaacactagggagaacaacaagtccacagaagtcacatgtctgttcattaaacgcacaggaagaccttgaactaaacccttcacaaaacatctaacacagagcttgcaatggtgaggagcctctctctcctgcacagccagtgaacaatctaggcttggagagacagagagaagagcaagagcattctaataagcaggtgtctgtgacctcctgagtaaccaaccgtgaaaccaagagataagtacagtcatgggtcactgaacaacgaggacacattttaagaattgcgttgttaggggattttgttttgggaacaccacggaagggacttacataaacccagatggtacaggcgactccacacctaggctctatggggcagcctgctgctcttggctacaaaccggcacaacatgtttactgaatgccttaggcaactgtaacacaacaagaaacatttgtatatataaacacaaaaaagtaaagtaaaaacacagtataaaaggtaaaaaatgggacactcgtctaggaaacatggagtttgcagaactggaagttgctctgggtgatcagggagcgagtggcgagtgaatgggaagacctaggacatgactgtccattaccacagacttcaccaacactgcacactcaggctacgctaaagttagaaaaaaacatttcctttcctctgtgataaattaactttagcttactgtaactttttttactttataaactttttaactttttgactcttttaataataccggtttaacacacaaatgtattgcacagctacacaaaagtattccttcttcatatccttactctatatgctgttttccaccttaaaaaaaaaaacaacctttaaaacttttttcttttttttt

SEQ ID NO: 14355 - RNA, 3549 nt, Homo sapiens
  source 1..3549: mol_type = other RNA
gctgggattacaggcatgagccaccgcgcccggcctgctctaacttattttaagaatcactgttctattctggaaagggaaaagaccaccaccaagaagggaaaggagaccatgctggacagcctaatagtctaacaggggatcctagggtgcctgagctcatgggagcaaaccttgttcaggcaccgcaagcccaacgcagcatgcagattgggaaggcgcaataatgcaaacaccatcaggaagaaagctatggatgatggaaaacactgtgtgctccacgtgacagaagggagccacctgatttgtcgcatcgggccagtgtaaggaagtgtaatttagtgggactgccagtgacactaagtcaggccttgatcagggtctggactcagtatggacacgagccactgggtgcagggggctcatgcctgccacctctctttttttcccttactatagagactttgatctgtccaccatttctatgtgagctttgggcttcctgtcacaggtctgttgtcaccgtggggccatgttggagtcggtagattttcagacagtgaagccacatgaagctgtgaatgctgatgtggctgctgcagagcccagtctctccccggtgcagggcctctgagacgacgggactgtcctcagatggttggaagaaatgggttatcttaggcagttaggaaaagagggacaggtgtcccaggatgtggaaaacttgagttcatcccctctcttccctccagcaaggatttcagtgctacatctaaaaagagaagccctgttgccgatttaataatttacagtctctaaatccaaaagggcctccatgtgctagtgagactcatgccctcagttatgttcacgatcttcctgagaagtcagacaatacaggtagaacaaaagatagtggttgtactttctcttctgcgtagtgtgggtaagagcatgcggtttgccgcatgcagtgttgttaatcttttgattgtgttgtgaatggctgaaaaaaaagctgaaagtttgattgaactgaaatccaatccatgtcaacataaggaatattctagtgagtttactgtcctaagagaaggtctctcctggggaacccctggtatgcagagctccctgggacttgcagattggacagagagggtgtgccaaaggggtataaacccttctgatggagagagtcgggcgtgtcttcattttggtagttctggaaaggctcctctttaaagattctgatttaataatgttcacttttgttaagattgaatatcattttgaaatcatttctaaacgtgtttcctttataggcactttatctattaaatttacagtggagccaaatgtattagcaaaatctccaagttgcaaaatgaatactcagaatcaaactatagattttttggtgatactttcagaaaaacaatttctttctaaagttgcaaatcatgaaagggaatgaaagtacattaacttgatttcttccctgtaattcaaacattcaacattcaaattaactttcataatttctcactttgtgacaagttgatttacgcatagttggtatttcattaatgcgatttatatagatggaattcttaaggataaacaaatgtttttgactattgcctggggttctttgggaatagatgctttctgaaaatttaaataagaacattactgttaaagccatgaatctagtttggagaacccactgcagttcattttacagagaaacaccttgtcaatggcatcttcatggtgtttactgaaggtaaaaggcaggatattaaatgtgagaactctctctccagctactgattctgcctgtctcgaattcaggtgagaatgacccatacagatacatggattgcacttgaatctgtgctctggtatttgtgtcatccggaggctgagaacgcctgttggtggtgtcgcagatggctctgctgtcttgtgtggacaaactgaaagggattcaggagcttcttctgtaattttactctgctgtttttcatggacatagtgaaagggatccaggagtttcttctgcaatttggctgtagttggactttgaaaaaaacttgaagagtgtgtgtgcgcgcgcgcgcgtgtgtgtgtgtgtttgaaaagagaattagaaaatgaaggtagacactgggtatgctcccccaggatgtggcgatggggcgcccggccgccctggctacacgtcgaaccagtggtcccccatgcagacgcggttccactcgcagccacagttccagcaccactcgagcctgcactggggctgcggacacttcatgtgcatgcagcctccatttttttccactggtacatggcagcggggacagggcttggtggttttcttgatggtttctttggaggctgcttcccaacgagcctgctcggcggctctttcatcgactctgtaggcctgagtagttgttcctgaggcttcaaatacggcactgcactccccttcatggtacgcttctttacattcccggcagaaggcaaacccacagcccaggccattgcccccttcgcaggtgactttcctctggtcaggctccggcagcagccccgctccacagccagggcgggggcataacacgccccccatctgcaggacacactcctctgcaccatactgctggtaccggttgtactgctcttctcccagaatcctgaagtgatggagctctttaatcaaggagttgggacagccagccacacaaggcagggagtagccaagttgagggtcgtgaacaaactgccgatcattgagtcttgtcacacagtataagtggaaacagtctaagcaaatcacgtggcgggagttgcactggaaaaccaggacggggctcctgacgtctgtgcacgtaatgcaagtgatgttccgactatttgttgcgatcaggtgcaaagctactgatgtttccttgtcagaggtggggtgtgctccacatttaaagaaaaattctgcactagtcccagggcagtgtggggattggcattcaccactcatccggtttggaattaaaacatcatcccagcaagatggaccctgggtcaaggtgagcgttgcctgcctgcaggtgctgcactgtaccctgagttttcccggctgcactctttgacaggggcctttgcaatacacataaaagctgttgtagattgatctacctggacttccagctggtggtgagtccttcctgctgtcagtgtgcagaatgacagccagccccacagagtctcctgggaggactgagctgctgaggtccacccgagtcaagctctggggctcccgctcacagcctcccgccgcgtttctggggtcgtcgcctccagttgcattcatttcttgaccttttctccacggtctctgcacaatgtgaacaatgctctgctgatccaggtcacaattctatcatggtcactgggtaggtggcggctgcgggccaggaacaggcccatgcgcgcagcggcgccagccgcgcctcccaccagcggctctcctgggttaaatcctcc

SEQ ID NO: 14356 - RNA, 3747 nt, Homo sapiens
  source 1..3747: mol_type = other RNA
gctgggattacaggcatgagccaccgcgcccggcctgctctaacttattttaagaatcactgttctattctggaaagggaaaagaccaccaccaagaagggaaaggagaccatgctggacagcctaatagtctaacaggggatcctagggtgcctgagctcatgggagcaaaccttgttcaggcaccgcaagcccaacgcagcatgcagattgggaaggcgcaataatgcaaacaccatcaggaagaaagctatggatgatggaaaacactgtgtgctccacgtgacagaagggagccacctgatttgtcgcatcgggccagtgtaaggaagtgtaatttagtgggactgccagtgacactaagtcaggccttgatcagggtctggactcagtatggacacgagccactgggtgcagggggctcatgcctgccacctctctttttttcccttactatagagactttgatctgtccaccatttctatgtgagctttgggcttcctgtcacaggtctgttgtcaccgtggggccatgttggagtcggtagattttcagacagtgaagccacatgaagctgtgaatgctgatgtggctgctgcagagcccagtctctccccggtgcagggcctctgagacgacgggactgtcctcagatggttggaagaaatgggttatcttaggcagttaggaaaagagggacaggtgtcccaggatgtggaaaacttgagttcatcccctctcttccctccagcaaggatttcagtgctacatctaaaaagagaagccctgttgccgatttaataatttacagtctctaaatccaaaagggcctccatgtgctagtgagactcatgccctcagttatgttcacgatcttcctgagaagtcagacaatacaggtagaacaaaagatagtggttgtactttctcttctgcgtagtgtgggtaagagcatgcggtttgccgcatgcagtgttgttaatcttttgattgtgttgtgaatggctgaaaaaaaagctgaaagtttgattgaactgaaatccaatccatgtcaacataaggaatattctagtgagtttactgtcctaagagaaggtctctcctggggaacccctggtatgcagagctccctgggacttgcagattggacagagagggtgtgccaaaggggtataaacccttctgatggagagagtcgggcgtgtcttcattttggtagttctggaaaggctcctctttaaagattctgatttaataatgttcacttttgttaagattgaatatcattttgaaatcatttctaaacgtgtttcctttataggcactttatctattaaatttacagtggagccaaatgtattagcaaaatctccaagttgcaaaatgaatactcagaatcaaactatagattttttggtgatactttcagaaaaacaatttctttctaaagttgcaaatcatgaaagggaatgaaagtacattaacttgatttcttccctgtaattcaaacattcaacattcaaattaactttcataatttctcactttgtgacaagttgatttacgcatagttggtatttcattaatgcgatttatatagatggaattcttaaggataaacaaatgtttttgactattgcctggggttctttgggaatagatgctttctgaaaatttaaataagaacattactgttaaagccatgaatctagtttggagaacccactgcagttcattttacagagaaacaccttgtcaatggcatcttcatggtgtttactgaaggtaaaaggcaggatattaaatgtgagaactctctctccagctactgattctgcctgtctcgaattcaggtgagaatgacccatacagatacatggattgcacttgaatctgtgctctggtatttgtgtcatccggaggctgagaacgcctgttggtggtgtcgcagatggctctgctgtcttgtgtggacaaactgaaagggattcaggagcttcttctgtaattttactctgctgtttttcatggacatagtgaaagggatccaggagtttcttctgcaatttggctgtagttggactttgaaaaaaacttgaagagtgtgtgtgcgcgcgcgcgcgtgtgtgtgtgtgtttgaaaagagaattagaaaatgaaggtagacactgggtatgctcccccaggatgtggcgatggggcgcccggccgccctggctacacgtcgaaccagtggtcccccatgcagacgcggttccactcgcagccacagttccagcaccactcgagcctgcactggggctgcggacacttcatgtgcatgcagcctccatttttttccactggtacatggcagcggggacagggcttggtggttttcttgatggtttctttggaggctgcttcccaacgagcctgctcggcggctctttcatcgactctgtaggcctgagtagttgttcctgaggcttcaaatacggcactgcactccccttcatggtacgcttctttacattcccggcagaaggcaaacccacagcccaggccattgcccccttcgcaggtgactttcctctggtcaggctccggcagcagccccgctccacagccagggcgggggcataacacgccccccatctgcaggacacactcctctgcaccatactgctggtaccggttgtactgctcttctcccagaatcctgaagtgatggagctctttaatcaaggagttgggacagccagccacacaaggcagggagtagccaagttgagggtcgtgaacaaactgccgatcattgagtcttgtcacacagtataagtggaaacagtctaagcaaatcacgtggcgggagttgcactggaaaaccaggacggggctcctgacgtctgtgcacgtaatgcaagtgatgttccgactatttgttgcgatcaggtgcaaagctactgatgtttccttgtcagaggtggggtgtgctccacatttaaagaaaaattctgcactagtcccagggcagtgtggggattggcattcaccactcatccggtttggaattaaaacatcatcccagcaagatggaccctgggtcaaggtgagcgttgcctgcctgcaggtgctgcactgtaccctgagttttcccggctgcactctttgacaggggcctttgcaatacacataaaagctgttgtagattgatctacctggacttccagctggtggtgagtccttcctgctgtcagtgtgcagaatgacagccagccccacagagtctcctgggaggactgagctgctgaggtccacccgagtcaagctctggggctcccgctcacagcctcccgccgcgtttctggggtcgtcgcctccagttgcattcatttcttgaccttttctccacggtctctgcacaatgtgaacaatgctctgctgatccaggtcacaattctgcacagtccagtcattcctcagctccttccctgcgaaaatcacacgcaactggtcagccggaaccccctgtcgcttagcaaccacctccttgagctggaagatgctggtgtcagaatcgacctccactgggaaaccatggctggagttgaacctgacaaacactatcatggtcactgggtaggtggcggctgcgggccaggaacaggcccatgcgcgcagcggcgccagccgcgcctcccaccagcggctctcctgggttaaatcctccaggcctccccgcccccgcgcccggccctaggaat

SEQ ID NO: 14357 - RNA, 3808 nt, Homo sapiens
  source 1..3808: mol_type = other RNA
gctgggattacaggcatgagccaccgcgcccggcctgctctaacttattttaagaatcactgttctattctggaaagggaaaagaccaccaccaagaagggaaaggagaccatgctggacagcctaatagtctaacaggggatcctagggtgcctgagctcatgggagcaaaccttgttcaggcaccgcaagcccaacgcagcatgcagattgggaaggcgcaataatgcaaacaccatcaggaagaaagctatggatgatggaaaacactgtgtgctccacgtgacagaagggagccacctgatttgtcgcatcgggccagtgtaaggaagtgtaatttagtgggactgccagtgacactaagtcaggccttgatcagggtctggactcagtatggacacgagccactgggtgcagggggctcatgcctgccacctctctttttttcccttactatagagactttgatctgtccaccatttctatgtgagctttgggcttcctgtcacaggtctgttgtcaccgtggggccatgttggagtcggtagattttcagacagtgaagccacatgaagctgtgaatgctgatgtggctgctgcagagcccagtctctccccggtgcagggcctctgagacgacgggactgtcctcagatggttggaagaaatgggttatcttaggcagttaggaaaagagggacaggtgtcccaggatgtggaaaacttgagttcatcccctctcttccctccagcaaggatttcagtgctacatctaaaaagagaagccctgttgccgatttaataatttacagtctctaaatccaaaagggcctccatgtgctagtgagactcatgccctcagttatgttcacgatcttcctgagaagtcagacaatacaggtagaacaaaagatagtggttgtactttctcttctgcgtagtgtgggtaagagcatgcggtttgccgcatgcagtgttgttaatcttttgattgtgttgtgaatggctgaaaaaaaagctgaaagtttgattgaactgaaatccaatccatgtcaacataaggaatattctagtgagtttactgtcctaagagaaggtctctcctggggaacccctggtatgcagagctccctgggacttgcagattggacagagagggtgtgccaaaggggtataaacccttctgatggagagagtcgggcgtgtcttcattttggtagttctggaaaggctcctctttaaagattctgatttaataatgttcacttttgttaagattgaatatcattttgaaatcatttctaaacgtgtttcctttataggcactttatctattaaatttacagtggagccaaatgtattagcaaaatctccaagttgcaaaatgaatactcagaatcaaactatagattttttggtgatactttcagaaaaacaatttctttctaaagttgcaaatcatgaaagggaatgaaagtacattaacttgatttcttccctgtaattcaaacattcaacattcaaattaactttcataatttctcactttgtgacaagttgatttacgcatagttggtatttcattaatgcgatttatatagatggaattcttaaggataaacaaatgtttttgactattgcctggggttctttgggaatagatgctttctgaaaatttaaataagaacattactgttaaagccatgaatctagtttggagaacccactgcagttcattttacagagaaacaccttgtcaatggcatcttcatggtgtttactgaaggtaaaaggcaggatattaaatgtgagaactctctctccagctactgattctgcctgtctcgaattcaggtgagaatgacccatacagatacatggattgcacttgaatctgtgctctggtatttgtgtcatccggaggctgagaacgcctgttggtggtgtcgcagatggctctgctgtcttgtgtggacaaactgaaagggattcaggagcttcttctgtaattttactctgctgtttttcatggacatagtgaaagggatccaggagtttcttctgcaatttggctgtagttggactttgaaaaaaacttgaagagtgtgtgtgcgcgcgcgcgcgtgtgtgtgtgtgtttgaaaagagaattagaaaatgaaggtagacactgggtatgctcccccaggatgtggcgatggggcgcccggccgccctggctacacgtcgaaccagtggtcccccatgcagacgcggttccactcgcagccacagttccagcaccactcgagcctgcactggggctgcggacacttcatgtgcatgcagcctccatttttttccactggtacatggcagcggggacagggcttggtggttttcttgatggtttctttggaggctgcttcccaacgagcctgctcggcggctctttcatcgactctgtaggcctgagtagttgttcctgaggcttcaaatacggcactgcactccccttcatggtacgcttctttacattcccggcagaaggcaaatgccaatgtgtccacgctgctcctcaggcaagccattctccccagtgcacagatgaggaaatcggggctctgagaggttaactgaccccacagcccaggccattgcccccttcgcaggtgactttcctctggtcaggctccggcagcagccccgctccacagccagggcgggggcataacacgccccccatctgcaggacacactcctctgcaccatactgctggtaccggttgtactgctcttctcccagaatcctgaagtgatggagctctttaatcaaggagttgggacagccagccacacaaggcagggagtagccaagttgagggtcgtgaacaaactgccgatcattgagtcttgtcacacagtataagtggaaacagtctaagcaaatcacgtggcgggagttgcactggaaaaccaggacggggctcctgacgtctgtgcacgtaatgcaagtgatgttccgactatttgttgcgatcaggtgcaaagctactgatgtttccttgtcagaggtggggtgtgctccacatttaaagaaaaattctgcactagtcccagggcagtgtggggattggcattcaccactcatccggtttggaattaaaacatcatcccagcaagatggaccctgggtcaaggtgagcgttgcctgcctgcaggtgctgcactgtaccctgagttttcccggctgcactctttgacaggggcctttgcaatacacataaaagctgttgtagattgatctacctgctggacttccagctggtggtgagtccttcctgctgtcagtgtgcagaatgacagccagccccacagagtctcctgggaggactgagctgctgaggtccacccgagtcaagctctggggctcccgctcacagcctcccgccgcgtttctggggtcgtcgcctccagttgcattcatttcttgaccttttctccacggtctctgcacaatgtgaacaatgctctgctgatccaggtcacaattctgcacagtccagtcattcctcagctccttccctgcgaaaatcacacgcaactggtcagccggaaccccctgtcgcttagcaaccacctccttgagctggaagatgctggtgtcagaatcgacctccactgggaaaccatggctggagttgaacctgacaaacactatcatggtcactgggtaggtggcggctgcgggccaggaacaggcccatgcgcgcagcggcgccagccgcgcctcccaccagcggctctcctgggttaaatcctccaggcct

SEQ ID NO: 14358 - RNA, 2535 nt, Homo sapiens
  source 1..2535: mol_type = other RNA
gctgggattacaggcatgagccaccgcgcccggcctgtgcttgggatttctttgcagttcgggtaagcgaggaggcaccgcaccaaccactgtgtgatttccgcccgacaagagcggcccaggagagcttcctacctccagccacactggttactcctctaaacctggaaggtacttttactgataaggaaggtggtgatcttttctctatcacatgtgggactggaatgttattataactgcactgaaaaaggcaaaggagctcagctctctgagagagagaattcaggcatgggaggtcagatggattgctgaaaatgctggttaagagcctcttacaaatctacctctttgcaagtctcttatctacctactaatcatcgaaaatccagaaagctcagggtttaggaccataatttgcaaaatctccgcaatcctgttggttgaaaagcacaggtgaaatatgaaatctcactcaagctcactgttaagtgaaccaaggacaaactgattttattacgtctatttcctaaaaagccttctccaataagccctcggtgaaggaagtggtatattctggagtatgcagaatttttattaacagcatttgcctctggaactgtggacacctctttgcaagtggagaccctgttttctcccattcctaacctaggggaagactccacaccctcagccatgctcatgcccccgggccaggagctgctgtggggggagcacacgcttcctcaaaatggccatttctgatcttgaccttcacgccacaattagcagtaagtaatgtgagtcttgctttatcccacagagggaatttccgtttggacaatgttttcagaaatgtaatcttttcaatatgaaactgctgatggaccaagaaaacaaaaccctcaacccaagggaacatcagattgctggtcaaggagaaatgaggagctgacggtctcagcatttatttgacttgctccacggacagagcaggagaaggctcaaacctcttcaccccaagactctccctcacacctgcctcctcacccaaaccctagaggacaggacaggaaccaccaacattttatggttttcaaaaatcctgcattgaacactgactgtgagccaggtgctgatggaagtgcctttcactcgatgatctcatctactgctcacaattccaccagttaaggcccacattttggacaaagagcctgaggaacctaccccctccccgcagtgctcacacttttgtccctccagaggacgggaacttcctctttctttagcaagctctgtaggggaccagcccacaggccctggggtagggcagcccgaccgcggcccttccctcaccatggcctatggttctccttcccttttcctttaagaaggccaggtgagaatcacaggaaagggagaatttattttgattaaaaataacatttcttaaagggggcatcgattttccctttccaaagtccaatcactcatccctatccggagcgacagaacctggggccggggctcaggcctcccacgcaggctgtgctcagtggacacaggaatggattcctgggacactgcggggggtggaggggcgtgatgcagggtccccacgatcagccgcagtctctctaacactgcaggtggtgccaagaggcaggcatgctcccagcacaagggacggtggcgcagaagaatacagagaagctcacaaaacatgccggcatgggctcaggagagctacgggggtagtggtggtactgctccctggtgcagggcagcagctgtgtctccccctgcctccctcccacccgagggccctgctcacctggccccagcttggagatggcatataagagatcatagtttatgactggggtcgcatcttccacttgtttccatcccactggcggagaggcgggaggggagatcagaaactgcttgtctggatttggcggagccaggtgtgagcttcctatgtgtaaggtctgagcaaaatataacttcatttcctttcccagaaactcagtcttatgcagctggagcctggcatctgctgcggagaaggggttgctgaagtttattctgactcgtttgaagctcttaaaatactgaaaggtgatgtccttgtcatacgtcctaaagagggactcaaatttggcccggcacaggccgtccacgaacacgcgcgggtccaggtgacaggcgatggtggcgctgggcaggtcctgcaggtccacctcctccatctcgcagtcaatgaagctccagtcgccgccgccctcgtccgcctcggccgcccccgagaggggcgcgaagggccgcagcgtcaccccgggccgcgctcgcgcctcggccgcctccgccgcctccgccgcggccccgagctggggaccggccacgccgtcctccatccccgcgcccgcgcgaccctgtgcgccccagcgggctgctccgggcttgcgcgccggagcctcacgcgctccggtccgcgcccggccggcggctccgccgttaaccccctcg

SEQ ID NO: 14359 - RNA, 2880 nt, Homo sapiens
  source 1..2880: mol_type = other RNA
gctgggattacaggcatgagccaccgcgcccggcctgtgcttgggatttctttgcagttcgggtaagcgaggaggcaccgcaccaaccactgtgtgatttccgcccgacaagagcggcccaggagagcttcctacctccagccacactggttactcctctaaacctggaaggtacttttactgataaggaaggtggtgatcttttctctatcacatgtgggactggaatgttattataactgcactgaaaaaggcaaaggagctcagctctctgagagagagaattcaggcatgggaggtcagatggattgctgaaaatgctggttaagagcctcttacaaatctacctctttgcaagtctcttatctacctactaatcatcgaaaatccagaaagctcagggtttaggaccataatttgcaaaatctccgcaatcctgttggttgaaaagcacaggtgaaatatgaaatctcactcaagctcactgttaagtgaaccaaggacaaactgattttattacgtctatttcctaaaaagccttctccaataagccctcggtgaaggaagtggtatattctggagtatgcagaatttttattaacagcatttgcctctggaactgtggacacctctttgcaagtggagaccctgttttctcccattcctaacctaggggaagactccacaccctcagccatgctcatgcccccgggccaggagctgctgtggggggagcacacgcttcctcaaaatggccatttctgatcttgaccttcacgccacaattagcagtaagtaatgtgagtcttgctttatcccacagagggaatttccgtttggacaatgttttcagaaatgtaatcttttcaatatgaaactgctgatggaccaagaaaacaaaaccctcaacccaagggaacatcagattgctggtcaaggagaaatgaggagctgacggtctcagcatttatttgacttgctccacggacagagcaggagaaggctcaaacctcttcaccccaagactctccctcacacctgcctcctcacccaaaccctagaggacaggacaggaaccaccaacattttatggttttcaaaaatcctgcattgaacactgactgtgagccaggtgctgatggaagtgcctttcactcgatgatctcatctactgctcacaattccaccagttaaggcccacattttggacaaagagcctgaggaacctaccccctccccgcagtgctcacacttttgtccctccagaggacgggaacttcctctttctttagcaagctctgtaggggaccagcccacaggccctggggtagggcagcccgaccgcggcccttccctcaccatggcctatggttctccttcccttttcctttaagaaggccaggtgagaatcacaggaaagggagaatttattttgattaaaaataacatttcttaaagggggcatcgattttccctttccaaagtccaatcactcatccctatccggagcgacagaacctggggccggggctcaggcctcccacgcaggctgtgctcagtggacacaggaatggattcctgggacactgcggggggtggaggggcgtgatgcagggtccccacgatcagccgcagtctctctaacactgcaggtggtgccaagaggcaggcatgctcccagcacaagggacggtggcgcagaagaatacagagaagctcacaaaacatgccggcatgggctcaggagagctacgggggtagtggtggtactgctccctggtgcagggcagcagctgtgtctccccctgcctccctcccacccgagggccctgctcacctggccccagcttggagatggcatataagagatcatagtttatgactggggtcgcatcttccacttgtttccatcccactggcggagaggcgggaggggagatcagaaactgcttgtctggatttggcggagccaggtgtgagcttcctatgtgtaaggtctgagcaaaatataacttcatttcctttcccagaaactcagtcttatgcagctggagcctggcatctgctgcggagaaggggttgctgaagtttattctgactcgtttgaagctcttaaaatactgaaaggtgatgtccttgtcatacgtcctaaagagggactcaaatttggccttggagaacctatggaaggcgcagtgtctctgcagtgggagcgaggattcaggataagagaggagagtgtcttcaggaatgttcactgctagcaagcgcggggaggcactggtggatgcctgctccacatggggctgcgggtaggagcagggtagtcggtccctgccaggcaggtcgttaaggagcagtcggaacaacctacgaccttgctctccttgcattccccggcttttcttcagtttagggacatttctgagactttcccacgagggatcccgcagaggcacgtgcgaaggaacgcggagctggcggacggtagagttcatctggccgcctctcactctttttccccacctctcttgagcacgggcaagtttctggcaaaagtgtgtcttcgtacatttggaattttgtatgacctcatcaataggcactgtgacccactgtttagttttgaagttatgattcagaatttgggagagatgactttgaagaatatttttagaatacaggttcagggcctggtttcactttcgctgaagatatcactgtttgccacacaggcaatcagggagctaaaactgtagttaaagtttctaaaatgcatcttgctttcttacagtgaaagcgctacagacccacgcagtcaagcccctagtgagattcctttccaagaggctgtaggttccttcttgagctggtgcttat

SEQ ID NO: 14360 - RNA, 3093 nt, Homo sapiens
  source 1..3093: mol_type = other RNA
gctgggattacaggcatgagccaccgcgcccggccttacccacattttaaagttaagaaaagtgatgcacttagagattaatgaatatgtcttaattcacatcactggtaagtggttaatctttattgacaaccttagtagcatggctcctgaacctgttcctaaccactgagccttattggctttatgaatgaatggttgcattataatgaatgagagaaggcttctaatactaaatagtcacgacatgcccatgaagctgaaatgaaagagaatagtgagaaggagaaaacataatctgaaagtttgtacacaaatgaaagtaatgcagtgtagaggccactcaactcagagcatttcactcaagaatgcatttgctcccactcgctttcttgcttccaagtctgctgattaaaattccatccaacttgaaagattttgtaaactattcccacttgtaaatatttgttctgtgttcttctcttctatatcctagtctacatgagagatggacttatgtctattttgtccatcactgtgtccctagcatctagaacagtgtttgtgaaagagtagacagtgacaaagttatttttattgtgttactatatttttgtatttatgtattacagaattttaagtgaatacaaatatacagaaaatatagtataacactccgttcccatcaaacagcttcaatgattactcactcagaaaacttcacttcaaatataatatgaccctctttctcccactcactgaattattttaaagcattctcagtcattatctcatctcatccatattttaaagaatttattttaattgaatgaaaactcatatcacatattacctctttcattaaatactgttgaatcctctcaatcaaaaaagaattttcccctatttgaaagtctgtgggattgtacacttcttttatttcaaaacctgttttgctgtgaatgtgttttgtgaacatgttttctaccagtttgagattccaagtccctgaaagattgggaaaatatctcatataactttgcgttccattcaaggtctattgcagtatcttgaatttggaaactagttttctgtcttctctgcaccacttccaagtacatggaaaagggtgctaaaatagtactctttctgtttccatttcagccaagaacaagggacaatagatggcatacacccctcactttcagtgaggtgctagacatgaaaagcagatgactgaaaccttgttttcagtcccacagtttgacatccaccttaattgaataaaaggattgaagttgaagagaacaaagcagggaacttgtttgaagaaagctgattgaactgctacggcattccctcattcattggtccagtcacaaagaatgatttcttctctcacttcttctttctcacttttgatccatcatctccccagctcgaaacctgccaactttttactatatcttctccattccagcagggaagtccatctgcagcagctaattcattagcacaaagctgatcagctagacctccatagaatgacctgtacagtcgaaggctgttgataaattcttttcttctgttggcaagcgtctcttcactgttccttgtggtggtcttcattccatgcttctctttgctctgatcaaaagaacaacgggggctttgtgtgggtgttcttacagggcggccacaaatcctatttacctgttccaataatttttgtccattgaggtgagcctgtaacacagcatcattaacaagcaagtgaaagttcagcagcacgtgtccaatgtcgtatgttccatgcattgcatccgagagttcttccaacgaccggatatatgcatgccagtgtggattaagctccgccatgtgcgccaggcagcctcgcatgacattgaggcagtatcccatacaaggcttagtgagcgccaggccttggcagtgcgggcagtattgcatcttcaggagggctctgctgcactctttggagaagtgcagatagtctgtggtgttgatgacttcaatgcccagattgagtgcctgcagaaaagtgcggctgggcagcagggacctccccatctgtcccattactctttggggaatattaccaaatggactcacatcccggcgagccatccggatgcattctgagtattccagggaactgtcagtcacaccagggttaatgaggtggttgtagaccagaggaaaaagactgtcaaaaaatctgtttacaaattcttcaggattaacatccgcaccaaataaatacagccccacatcagtgaagaactcctgaaccgaagcagcagcctccaaggccatgttcctgtaggtactgcaaaaaagtatactggtgtaattttctgcttgtttgatgagagtttcaagggtttcttgaaaagcagccgcatttcgagatattagaaactttaatgtagagctggacgtttgaagaaactgctgcatatcctggcgagccgcaatctgatatctctcctccatcttcctggtgcaacatgtaggctttttggatatgcaaacctgaagatcaggtcctgcccgcggcgaatccggcagccccctgacagctcccagcagccgccactggaaaagtttccgaacttcttcgcaggtctgcacgccctcgctgcgggcggacccaaccagggccagaaggaggaggcagcgaaagcccacgggccaggtctgtgcgtccatcctcgccgtcctggtcccctttacccgccagtggaccccactcgccctgcgcgccctggctgagctgcagacgtggaagacacagcggccgaggctctcgagcggtgcgagccggctgcggggtgtacggaccgcccgcgggcaccggcttcacctgggagcagttagctcttcccggaggaggccctaagctgagacaccagagttttccagctgagcaccctctggtcttcttccctagccgagaagagtgggcggctgggcggggcgaagaaaactagtggagccgcagggagcccgcaagcatccgctctggccaccactgctgcaactgctgccgctgccgccactgccgccact

SEQ ID NO: 14361 - RNA, 3135 nt, Homo sapiens
  source 1..3135: mol_type = other RNA
gctgggattacaggcatgagccaccgcgcccggccttacccacattttaaagttaagaaaagtgatgcacttagagattaatgaatatgtcttaattcacatcactggtaagtggttaatctttattgacaaccttagtagcatggctcctgaacctgttcctaaccactgagccttattggctttatgaatgaatggttgcattataatgaatgagagaaggcttctaatactaaatagtcacgacatgcccatgaagctgaaatgaaagagaatagtgagaaggagaaaacataatctgaaagtttgtacacaaatgaaagtaatgcagtgtagaggccactcaactcagagcatttcactcaagaatgcatttgctcccactcgctttcttgcttccaagtctgctgattaaaattccatccaacttgaaagattttgtaaactattcccacttgtaaatatttgttctgtgttcttctcttctatatcctagtctacatgagagatggacttatgtctattttgtccatcactgtgtccctagcatctagaacagtgtttgtgaaagagtagacagtgacaaagttatttttattgtgttactatatttttgtatttatgtattacagaattttaagtgaatacaaatatacagaaaatatagtataacactccgttcccatcaaacagcttcaatgattactcactcagaaaacttcacttcaaatataatatgaccctctttctcccactcactgaattattttaaagcattctcagtcattatctcatctcatccatattttaaagaatttattttaattgaatgaaaactcatatcacatattacctctttcattaaatactgttgaatcctctcaatcaaaaaagaattttcccctatttgaaagtctgtgggattgtacacttcttttatttcaaaacctgttttgctgtgaatgtgttttgtgaacatgttttctaccagtttgagattccaagtccctgaaagattgggaaaatatctcatataactttgcgttccattcaaggtctattgcagtatcttgaatttggaaactagttttctgtcttctctgcaccacttccaagtacatggaaaagggtgctaaaatagtactctttctgtttccatttcagccaagaacaagggacaatagatggcatacacccctcactttcagtgaggtgctagacatgaaaagcagatgactgaaaccttgttttcagtcccacagtttgacatccaccttaattgaataaaaggattgaagttgaagagaacaaagcagggaacttgtttgaagaaagctgattgaactgctacggcattccctcattcattggtcctaggtgagagaagtgttgaaggatccttggagctggaaggacagtcacaaagaatgatttcttctctcacttcttctttctcacttttgatccatcatctccccagctcgaaacctgccaactttttactatatcttctccattccagcagggaagtccatctgcagcagctaattcattagcacaaagctgatcagctagacctccatagaatgacctgtacagtcgaaggctgttgataaattcttttcttctgttggcaagcgtctcttcactgttccttgtggtggtcttcattccatgcttctctttgctctgatcaaaagaacaacgggggctttgtgtgggtgttcttacagggcggccacaaatcctatttacctgttccaataatttttgtccattgaggtgagcctgtaacacagcatcattaacaagcaagtgaaagttcagcagcacgtgtccaatgtcgtatgttccatgcattgcatccgagagttcttccaacgaccggatatatgcatgccagtgtggattaagctccgccatgtgcgccaggcagcctcgcatgacattgaggcagtatcccatacaaggcttagtgagcgccaggccttggcagtgcgggcagtattgcatcttcaggagggctctgctgcactctttggagaagtgcagatagtctgtggtgttgatgacttcaatgcccagattgagtgcctgcagaaaagtgcggctgggcagcagggacctccccatctgtcccattactctttggggaatattaccaaatggactcacatcccggcgagccatccggatgcattctgagtattccagggaactgtcagtcacaccagggttaatgaggtggttgtagaccagaggaaaaagactgtcaaaaaatctgtttacaaattcttcaggattaacatccgcaccaaataaatacagccccacatcagtgaagaactcctgaaccgaagcagcagcctccaaggccatgttcctgtaggtactgcaaaaaagtatactggtgtaattttctgcttgtttgatgagagtttcaagggtttcttgaaaagcagccgcatttcgagatattagaaactttaatgtagagctggacgtttgaagaaactgctgcatatcctggcgagccgcaatctgatatctctcctccatcttcctggtgcaacatgtaggctttttggatatgcaaacctgaagatcaggtcctgcccgcggcgaatccggcagccccctgacagctcccagcagccgccactggaaaagtttccgaacttcttcgcaggtctgcacgccctcgctgcgggcggacccaaccagggccagaaggaggaggcagcgaaagcccacgggccaggtctgtgcgtccatcctcgccgtcctggtcccctttacccgccagtggaccccactcgccctgcgcgccctggctgagctgcagacgtggaagacacagcggccgaggctctcgagcggtgcgagccggctgcggggtgtacggaccgcccgcgggcaccggcttcacctgggagcagttagctcttcccggaggaggccctaagctgagacaccagagttttccagctgagcaccctctggtcttcttccctagccgagaagagtgggcggctgggcggggcgaagaaaactagtggagccgcagggagcccgcaagcatccgctctggccaccactgctgcaactgctgccgctgccgccactgccgccact

SEQ ID NO: 14362 - RNA, 3208 nt, Homo sapiens
  source 1..3208: mol_type = other RNA
gctgggattacaggcatgagccaccgcgcccggccttacccacattttaaagttaagaaaagtgatgcacttagagattaatgaatatgtcttaattcacatcactggtaagtggttaatctttattgacaaccttagtagcatggctcctgaacctgttcctaaccactgagccttattggctttatgaatgaatggttgcattataatgaatgagagaaggcttctaatactaaatagtcacgacatgcccatgaagctgaaatgaaagagaatagtgagaaggagaaaacataatctgaaagtttgtacacaaatgaaagtaatgcagtgtagaggccactcaactcagagcatttcactcaagaatgcatttgctcccactcgctttcttgcttccaagtctgctgattaaaattccatccaacttgaaagattttgtaaactattcccacttgtaaatatttgttctgtgttcttctcttctatatcctagtctacatgagagatggacttatgtctattttgtccatcactgtgtccctagcatctagaacagtgtttgtgaaagagtagacagtgacaaagttatttttattgtgttactatatttttgtatttatgtattacagaattttaagtgaatacaaatatacagaaaatatagtataacactccgttcccatcaaacagcttcaatgattactcactcagaaaacttcacttcaaatataatatgaccctctttctcccactcactgaattattttaaagcattctcagtcattatctcatctcatccatattttaaagaatttattttaattgaatgaaaactcatatcacatattacctctttcattaaatactgttgaatcctctcaatcaaaaaagaattttcccctatttgaaagtctgtgggattgtacacttcttttatttcaaaacctgttttgctgtgaatgtgttttgtgaacatgttttctaccagtttgagattccaagtccctgaaagattgggaaaatatctcatataactttgcgttccattcaaggtctattgcagtatcttgaatttggaaactagttttctgtcttctctgcaccacttccaagtacatggaaaagggtgctaaaatagtactctttctgtttccatttcagccaagaacaagggacaatagatggcatacacccctcactttcagtgaggtgctagacatgaaaagcagatgactgaaaccttgttttcagtcccacagtttgacatccaccttaattgaataaaaggattgaagttgaagagaacaaagcagggaacttgtttgaagaaagctgattgaactgctacggcattccctcattcattggtcctaggtgagagaagtgttgaaggatccttggagctggaaggactaaaagggctggtagttggcctatgcctacgcaaatggaaggcagcccattcttgtagcagaagttggctgtcagtcacaaagaatgatttcttctctcacttcttctttctcacttttgatccatcatctccccagctcgaaacctgccaactttttactatatcttctccattccagcagggaagtccatctgcagcagctaattcattagcacaaagctgatcagctagacctccatagaatgacctgtacagtcgaaggctgttgataaattcttttcttctgttggcaagcgtctcttcactgttccttgtggtggtcttcattccatgcttctctttgctctgatcaaaagaacaacgggggctttgtgtgggtgttcttacagggcggccacaaatcctatttacctgttccaataatttttgtccattgaggtgagcctgtaacacagcatcattaacaagcaagtgaaagttcagcagcacgtgtccaatgtcgtatgttccatgcattgcatccgagagttcttccaacgaccggatatatgcatgccagtgtggattaagctccgccatgtgcgccaggcagcctcgcatgacattgaggcagtatcccatacaaggcttagtgagcgccaggccttggcagtgcgggcagtattgcatcttcaggagggctctgctgcactctttggagaagtgcagatagtctgtggtgttgatgacttcaatgcccagattgagtgcctgcagaaaagtgcggctgggcagcagggacctccccatctgtcccattactctttggggaatattaccaaatggactcacatcccggcgagccatccggatgcattctgagtattccagggaactgtcagtcacaccagggttaatgaggtggttgtagaccagaggaaaaagactgtcaaaaaatctgtttacaaattcttcaggattaacatccgcaccaaataaatacagccccacatcagtgaagaactcctgaaccgaagcagcagcctccaaggccatgttcctgtaggtactgcaaaaaagtatactggtgtaattttctgcttgtttgatgagagtttcaagggtttcttgaaaagcagccgcatttcgagatattagaaactttaatgtagagctggacgtttgaagaaactgctgcatatcctggcgagccgcaatctgatatctctcctccatcttcctggtgcaacatgtaggctttttggatatgcaaacctgaagatcaggtcctgcccgcggcgaatccggcagccccctgacagctcccagcagccgccactggaaaagtttccgaacttcttcgcaggtctgcacgccctcgctgcgggcggacccaaccagggccagaaggaggaggcagcgaaagcccacgggccaggtctgtgcgtccatcctcgccgtcctggtcccctttacccgccagtggaccccactcgccctgcgcgccctggctgagctgcagacgtggaagacacagcggccgaggctctcgagcggtgcgagccggctgcggggtgtacggaccgcccgcgggcaccggcttcacctgggagcagttagctcttcccggaggaggccctaagctgagacaccagagttttccagctgagcaccctctggtcttcttccctagccgagaagagtgggcggctgggcggggcgaagaaaactagtggagccgcagggagcccgcaagcatccgctctggccaccactgctgcaactgctgccgctgccgccactgccgccact

SEQ ID NO: 14363 - RNA, 3479 nt, Homo sapiens
  source 1..3479: mol_type = other RNA
gctgggattacaggcatgagccaccgcgcccggccttacccacattttaaagttaagaaaagtgatgcacttagagattaatgaatatgtcttaattcacatcactggtaagtggttaatctttattgacaaccttagtagcatggctcctgaacctgttcctaaccactgagccttattggctttatgaatgaatggttgcattataatgaatgagagaaggcttctaatactaaatagtcacgacatgcccatgaagctgaaatgaaagagaatagtgagaaggagaaaacataatctgaaagtttgtacacaaatgaaagtaatgcagtgtagaggccactcaactcagagcatttcactcaagaatgcatttgctcccactcgctttcttgcttccaagtctgctgattaaaattccatccaacttgaaagattttgtaaactattcccacttgtaaatatttgttctgtgttcttctcttctatatcctagtctacatgagagatggacttatgtctattttgtccatcactgtgtccctagcatctagaacagtgtttgtgaaagagtagacagtgacaaagttatttttattgtgttactatatttttgtatttatgtattacagaattttaagtgaatacaaatatacagaaaatatagtataacactccgttcccatcaaacagcttcaatgattactcactcagaaaacttcacttcaaatataatatgaccctctttctcccactcactgaattattttaaagcattctcagtcattatctcatctcatccatattttaaagaatttattttaattgaatgaaaactcatatcacatattacctctttcattaaatactgttgaatcctctcaatcaaaaaagaattttcccctatttgaaagtctgtgggattgtacacttcttttatttcaaaacctgttttgctgtgaatgtgttttgtgaacatgttttctaccagtttgagattccaagtccctgaaagattgggaaaatatctcatataactttgcgttccattcaaggtctattgcagtatcttgaatttggaaactagttttctgtcttctctgcaccacttccaagtacatggaaaagggtgctaaaatagtactctttctgtttccatttcagccaagaacaagggacaatagatggcatacacccctcactttcagtgaggtgctagacatgaaaagcagatgactgaaaccttgttttcagtcccacagtttgacatccaccttaattgaataaaaggattgaagttgaagagaacaaagcagggaacttgtttgaagaaagctgattgaactgctacggcattccctcattcattggtcctaggtgagagaagtgttgaaggatccttggagctggaaggactaaaagggctggtagttggcctatgcctacgcaaatggaaggcagcccattcttgtagcagaagttggctgtctagtggcagagtaaagagaggcagctgcattaggtgtaggctgtacttccaccaaaagtagaaaagagagggaaggtttctatgggctagaatagatgatatgggagaaaaggaacccaccaaaagatctcagcagaaagaggccaaaacattaccatcacatggagaaatagaggggagagacattgtcttaagcacacaaaagcactagggcatcagctgttaatacctgccaggctagaaaacatcaatgagagatcataaaattaccagtcacaaagaatgatttcttctctcacttcttctttctcacttttgatccatcatctccccagctcgaaacctgccaactttttactatatcttctccattccagcagggaagtccatctgcagcagctaattcattagcacaaagctgatcagctagacctccatagaatgacctgtacagtcgaaggctgttgataaattcttttcttctgttggcaagcgtctcttcactgttccttgtggtggtcttcattccatgcttctctttgctctgatcaaaagaacaacgggggctttgtgtgggtgttcttacagggcggccacaaatcctatttacctgttccaataatttttgtccattgaggtgagcctgtaacacagcatcattaacaagcaagtgaaagttcagcagcacgtgtccaatgtcgtatgttccatgcattgcatccgagagttcttccaacgaccggatatatgcatgccagtgtggattaagctccgccatgtgcgccaggcagcctcgcatgacattgaggcagtatcccatacaaggcttagtgagcgccaggccttggcagtgcgggcagtattgcatcttcaggagggctctgctgcactctttggagaagtgcagatagtctgtggtgttgatgacttcaatgcccagattgagtgcctgcagaaaagtgcggctgggcagcagggacctccccatctgtcccattactctttggggaatattaccaaatggactcacatcccggcgagccatccggatgcattctgagtattccagggaactgtcagtcacaccagggttaatgaggtggttgtagaccagaggaaaaagactgtcaaaaaatctgtttacaaattcttcaggattaacatccgcaccaaataaatacagccccacatcagtgaagaactcctgaaccgaagcagcagcctccaaggccatgttcctgtaggtactgcaaaaaagtatactggtgtaattttctgcttgtttgatgagagtttcaagggtttcttgaaaagcagccgcatttcgagatattagaaactttaatgtagagctggacgtttgaagaaactgctgcatatcctggcgagccgcaatctgatatctctcctccatcttcctggtgcaacatgtaggctttttggatatgcaaacctgaagatcaggtcctgcccgcggcgaatccggcagccccctgacagctcccagcagccgccactggaaaagtttccgaacttcttcgcaggtctgcacgccctcgctgcgggcggacccaaccagggccagaaggaggaggcagcgaaagcccacgggccaggtctgtgcgtccatcctcgccgtcctggtcccctttacccgccagtggaccccactcgccctgcgcgccctggctgagctgcagacgtggaagacacagcggccgaggctctcgagcggtgcgagccggctgcggggtgtacggaccgcccgcgggcaccggcttcacctgggagcagttagctcttcccggaggaggccctaagctgagacaccagagttttccagctgagcaccctctggtcttcttccctagccgagaagagtgggcggctgggcggggcgaagaaaactagtggagccgcagggagcccgcaagcatccgctctggccaccactgctgcaactgctgccgctgccgccactgccgccact

SEQ ID NO: 14364 - RNA, 4283 nt, Homo sapiens
  source 1..4283: mol_type = other RNA
gctgggattacaggcatgagccaccgcgcccggccttcctggtagtttccattccatctccctgtatttttctcttatcactctcgaagtctatctttcttgttcttttcctccctagctttttttttttaaacactcctttcaagctgtgtccaacacccacaaggaatgactatttttaactaatcttactgacctcatttaatctattcaataaaacctctgccctaaggagcaaagaaacttgcagaggaagtaaggcaaactggaagaagcatactgtcagcggattaaattcttgagcaaggcaatactccttatggattcttcccatgtacaatccgtaactcttcccatgggcctttatatcaaccctaagataattacactcctgcctcaaaataaaataaaataaaacccaccacatcttgtattgtagacatcccagctgcatgttaagctgagtgaaagtaccatgctgtcttttaaatcactttatatctacttaatcatcccacagtaacccgagttgaagaagttactttggtttctcataaatgaatatgcacgtgctgaacatatcggaaagaaccacaccctctcactgatgaacacgttggcagttctcccaactgttttatcaagagaagctagaaggtaaagaaaaggaaacagagccctataggaaaaatgattgacttcacacgtttgagcgatttgggcttcagctatgactttgctggagtacagatgggtgccatcagagcacaaagctgagcaaacctctcttcttaccctgtgccctccctgaatttttggatttctgagcttgtctactaccaacaaatgttttaccctccagtgcacctttgacagtatacagctctatttttcaaacggcaagtatgttatccaagttcagagatgcaactgaggaattaacatgaaaaccatctttcactcaataaatcagaagctgctagttaagtaagcctcaagaacctaagaaaaaacaccaaagtgtaagtattactcagtcaccaatctaaagacagaactttgactcaaggtagaaatgaaaccgtaattatataaatatatttataaatatttatacaattatatacttatacataagcacttacacagacttagaaaaaaatttaagaacattaattcaaaaggactcactgaagaataaacagatttttccatgatttccttgaggagatataaaactcattctttagggagagttcctcaaaattcaaccattagaaaccatatcctataactgtgtactagcaacacatggcatctttttttcttcttttcccaaatcccctaattgccaagagagcaatcttaaagtagatgaaaacctaaaggtctctacgcaacatctgaggaacatacgctcctcagataaaagaatcaatctaaatcctcaactgacaaaaaggtccatttaatatttttcattttacaagttaaaagttctagttttgccaccagaatcacgactacccccccttcagaggactccatttaagctcaaaatacgaaatgagcatagggtgaagttgatgtgtaaatggtattctacagattcaagatggcctcttctaaaaacactgaagaaagctttcaccaactctaatttgattttgggttttgttggcagaaaaagcccaagacatctgaaaattactagtaacctccgccatcctccttactaaatgttgtcttctgaatggagttgaaaggtcttccccttagagaggctttccgttttgataccttttgaaagaaaacagcatgcggactcatgttcaattcagtcaccagagccttttagagactattccaaccaggggcaaaaaatgaaccattatttctaaccaaaagaacatggttagcaactctcagctgaatggttttctttttccccagggacatacctaagtatgcctgaaacaacacaggacaatcaataaccatagtggttacaattccaagccattgtactacatgattattgaccagctgccttcctacagatcactgcagactcagacaatggagggctccaaaggaactaatatgctgtgctggcaaaaatagcaagcaccttcctatcccagtcaccacgataggttcacttcatgtccattcttggactagcaggatcaatacagagtaataaggaaaactgtctcaggttaggacaatgaaagtcaccccatgctatatgctccatatttaacactcattctgccaataacacatgtcatggaaatagtccttatagctgggaacatgaaaatcctttgaaaaaggtttttaagtatgatgagcaatcattacaagggatgctttttccacgtaaacaaaagcctggatattttgttaagcgacatttccacatgaagaacacaacaaaaccaaacccatgttagagaatttcttctccctgctaaacacggggacttacaaaaaagggagggttgttcttactctgaatctagccattcctttgcccgaagagtctggggagtaacgttaacatttgatcccaaaaaagtgccgtgcaagagaccacttactggaacacacaattcctgctgctagtactaggagaggtcttatccttacacttcagtttggtcaccagattaggtaagaaagaaaagtgtggggggagggggaggcagaagggtacggagtggggagcgagaaaacagaagaggagaaagaaacaaagggggagaaagagactgattataggagagatcaagaaataagagaaggaaggtgacttgcttgcccaactttggctctgtggtcctatgagccaaaatgcatacttagtgacatgtatctcacaggaaaagggaaaaaaggggtaagctgagagaggtcaagccatggtgttaatttctttcctgtacaaagacagtctcttgaggacaaaggcctgcctcttgcaatgtaatatcatagtccagatgagataatttccttcgaggaaagttggtgagaagttcaaaacgttcatttgggtatcctttagactgcacgtgcttcaccaaagctagcagtttagcttgctctggaagagtgatctgttccctttttccatctggataccgcaacatcagctgtgcttttggtccatttacatctatcccctccactactccatctgctttttcaggtggcatctccagtatctctgaatccacagctggcaatccttggtggtttgtggctgttccaggatcagttctgactggtggctcagtcagcggccttctattctcctcttttctatgccccaaatctttgtggggagactttctggacttggcaagattctctacctcttcttcttcatcagagccacaaacggatatgaactcctcactgccagaaaaaagttcagattcagattcttcatctgagcggctatcctgttttgtctgtgttgaatcaaaatgtgtttcttgtaaggaggctctgatggcagcttctagctggctgtcttcacttgcatctataaggctctctgaacgggcacattttttggggggactgctagaaagtccatccagttgtccatgttcacccagaaatcccgtcacttggtccaagaaagaagatacatctaactggtgccattctactagcttctgacctgtccgtgggtccaatatggaaacataggggaaatcccctaacttataaaactgtatgtatctctgaccttcctcactgtcatgataaacctgccagaaaatgaaatgttcccggataatattcttcacagcttcgttgctccacacatcgcggttgaggcactgacatgcaaagtcttgaacattttgaatgtttatcatcagccacttattttgcatctggccacactctttggctgtttcaaagctgcctttatgcatcaaatcaatgggtggccggaatagatctgcaagggtagttaatttcttatcgatagctcctccatttcttaattcttgttcttgccgaatagtttcagtctgaaaatcccggaaaccatcaaaaattgaacgtgcaggccgtcgtcttttaggagcaccaaataatggttctggttccaccagtatttcctgcttttgaggaattggggcacgaacttcttctcggtaatggtggtgaactgttgaattaaccccttcagcgccgaggacgccgcggagcccccgtgggcagccatcttaccgccgccgccgccgccgaacaac

SEQ ID NO: 14365 - RNA, 4426 nt, Homo sapiens
  source 1..4426: mol_type = other RNA
gctgggattacaggcatgagccaccgcgcccggccttcctggtagtttccattccatctccctgtatttttctcttatcactctcgaagtctatctttcttgttcttttcctccctagctttttttttttaaacactcctttcaagctgtgtccaacacccacaaggaatgactatttttaactaatcttactgacctcatttaatctattcaataaaacctctgccctaaggagcaaagaaacttgcagaggaagtaaggcaaactggaagaagcatactgtcagcggattaaattcttgagcaaggcaatactccttatggattcttcccatgtacaatccgtaactcttcccatgggcctttatatcaaccctaagataattacactcctgcctcaaaataaaataaaataaaacccaccacatcttgtattgtagacatcccagctgcatgttaagctgagtgaaagtaccatgctgtcttttaaatcactttatatctacttaatcatcccacagtaacccgagttgaagaagttactttggtttctcataaatgaatatgcacgtgctgaacatatcggaaagaaccacaccctctcactgatgaacacgttggcagttctcccaactgttttatcaagagaagctagaaggtaaagaaaaggaaacagagccctataggaaaaatgattgacttcacacgtttgagcgatttgggcttcagctatgactttgctggagtacagatgggtgccatcagagcacaaagctgagcaaacctctcttcttaccctgtgccctccctgaatttttggatttctgagcttgtctactaccaacaaatgttttaccctccagtgcacctttgacagtatacagctctatttttcaaacggcaagtatgttatccaagttcagagatgcaactgaggaattaacatgaaaaccatctttcactcaataaatcagaagctgctagttaagtaagcctcaagaacctaagaaaaaacaccaaagtgtaagtattactcagtcaccaatctaaagacagaactttgactcaaggtagaaatgaaaccgtaattatataaatatatttataaatatttatacaattatatacttatacataagcacttacacagacttagaaaaaaatttaagaacattaattcaaaaggactcactgaagaataaacagatttttccatgatttccttgaggagatataaaactcattctttagggagagttcctcaaaattcaaccattagaaaccatatcctataactgtgtactagcaacacatggcatctttttttcttcttttcccaaatcccctaattgccaagagagcaatcttaaagtagatgaaaacctaaaggtctctacgcaacatctgaggaacatacgctcctcagataaaagaatcaatctaaatcctcaactgacaaaaaggtccatttaatatttttcattttacaagttaaaagttctagttttgccaccagaatcacgactacccccccttcagaggactccatttaagctcaaaatacgaaatgagcatagggtgaagttgatgtgtaaatggtattctacagattcaagatggcctcttctaaaaacactgaagaaagctttcaccaactctaatttgattttgggttttgttggcagaaaaagcccaagacatctgaaaattactagtaacctccgccatcctccttactaaatgttgtcttctgaatggagttgaaaggtcttccccttagagaggctttccgttttgataccttttgaaagaaaacagcatgcggactcatgttcaattcagtcaccagagccttttagagactattccaaccaggggcaaaaaatgaaccattatttctaaccaaaagaacatggttagcaactctcagctgaatggttttctttttccccagggacatacctaagtatgcctgaaacaacacaggacaatcaataaccatagtggttacaattccaagccattgtactacatgattattgaccagctgccttcctacagatcactgcagactcagacaatggagggctccaaaggaactaatatgctgtgctggcaaaaatagcaagcaccttcctatcccagtcaccacgataggttcacttcatgtccattcttggactagcaggatcaatacagagtaataaggaaaactgtctcaggttaggacaatgaaagtcaccccatgctatatgctccatatttaacactcattctgccaataacacatgtcatggaaatagtccttatagctgggaacatgaaaatcctttgaaaaaggtttttaagtatgatgagcaatcattacaagggatgctttttccacgtaaacaaaagcctggatattttgttaagcgacatttccacatgaagaacacaacaaaaccaaacccatgttagagaatttcttctccctgctaaacacggggacttacaaaaaagggagggttgttcttactctgaatctagccattcctttgcccgaagagtctggggagtaacgttaacatttgatcccaaaaaagtgccgtgcaagagaccacttactggaacacacaattcctgctgctagtactaggagaggtcttatccttacacttcagtttggtcaccagattaggtaagaaagaaaagtgtggggggagggggaggcagaagggtacggagtggggagcgagaaaacagaagaggagaaagaaacaaagggggagaaagagactgattataggagagatcaagaaataagagaaggaaggtgacttgcttgcccaactttggctctgtggtcctatgagccaaaatgcatacttagtgacatgtatctcacaggaaaagggaaaaaaggggtaagctgagagaggtcaagccatggtgttaatttctttcctgtacaaagacagtctcttgaggacaaaggcctgcctcttgcaatgtaatatcatagtccagatgagataatttccttcgaggaaagttggtgagaagttcaaaacgttcatttgggtatcctttagactgcacgtgcttcaccaaagctagcagtttagcttgctctggaagagtgatctgttccctttttccatctggataccgcaacatcagctgtgcttttggtccatttacatctatcccctccactactccatctgctttttcaggtggcatctccagtatctctgaatccacagctggcaatccttggtggtttgtggctgttccaggatcagttctgactggtggctcagtcagcggccttctattctcctcttttctatgccccaaatctttgtggggagactttctggacttggcaagattctctacctcttcttcttcatcagagccacaaacggatatgaactcctcactgccagaaaaaagttcagattcagattcttcatctgagcggctatcctgttttgtctgtgttgaatcaaaatgtgtttcttgtaaggaggctctgatggcagcttctagctggctgtcttcacttgcatctataaggctctctgaacgggcacattttttggggggactgctagaaagtccatccagttgtccatgttcacccagaaatcccgtcacttggtccaagaaagaagatacatctaactggtgccattctactagcttctgacctgtccgtgggtccaatatggaaacataggggaaatcccctaacttataaaactgtatgtatctctgaccttcctcactgtcatgataaacctgccagaaaatgaaatgttcccggataatattcttcacagcttcgttgctccacacatcgcggttgaggcactgacatgcaaagtcttgaacattttgaatgtttatcatcagccacttattttgcatctggccacactctttggctgtttcaaagctgcctttatgcatcaaatcaatgggtggccggaatagatctgcaagggtagttaatttcttatcgatagctcctccatttcttaattcttgttcttgccgaatagtttcagtctgaaaatcccggaaaccatcaaaaattgaacgtgcaggccgtcgtcttttaggagcaccaaataatggttctggttccaccagtatttcctgcttttgaggaattggggcacgaacttcttcttctgtgtgtggtctgacagtagagacacttgctgaactggtactgggctcttcagcgattcctccaccatccaaaaacatagtgactgccatttccagattattgttgcacgcttcaagcatatgttttcctacactttcacttgcacaaatctattttcttgtgttgagttcgttctgtttctctctgaaaggtagatttttgaaatgcaaaagcatgaaactaacttctttttctcccaggt

SEQ ID NO: 14366 - RNA, 4431 nt, Homo sapiens
  source 1..4431: mol_type = other RNA
gctgggattacaggcatgagccaccgcgcccggccttcctggtagtttccattccatctccctgtatttttctcttatcactctcgaagtctatctttcttgttcttttcctccctagctttttttttttaaacactcctttcaagctgtgtccaacacccacaaggaatgactatttttaactaatcttactgacctcatttaatctattcaataaaacctctgccctaaggagcaaagaaacttgcagaggaagtaaggcaaactggaagaagcatactgtcagcggattaaattcttgagcaaggcaatactccttatggattcttcccatgtacaatccgtaactcttcccatgggcctttatatcaaccctaagataattacactcctgcctcaaaataaaataaaataaaacccaccacatcttgtattgtagacatcccagctgcatgttaagctgagtgaaagtaccatgctgtcttttaaatcactttatatctacttaatcatcccacagtaacccgagttgaagaagttactttggtttctcataaatgaatatgcacgtgctgaacatatcggaaagaaccacaccctctcactgatgaacacgttggcagttctcccaactgttttatcaagagaagctagaaggtaaagaaaaggaaacagagccctataggaaaaatgattgacttcacacgtttgagcgatttgggcttcagctatgactttgctggagtacagatgggtgccatcagagcacaaagctgagcaaacctctcttcttaccctgtgccctccctgaatttttggatttctgagcttgtctactaccaacaaatgttttaccctccagtgcacctttgacagtatacagctctatttttcaaacggcaagtatgttatccaagttcagagatgcaactgaggaattaacatgaaaaccatctttcactcaataaatcagaagctgctagttaagtaagcctcaagaacctaagaaaaaacaccaaagtgtaagtattactcagtcaccaatctaaagacagaactttgactcaaggtagaaatgaaaccgtaattatataaatatatttataaatatttatacaattatatacttatacataagcacttacacagacttagaaaaaaatttaagaacattaattcaaaaggactcactgaagaataaacagatttttccatgatttccttgaggagatataaaactcattctttagggagagttcctcaaaattcaaccattagaaaccatatcctataactgtgtactagcaacacatggcatctttttttcttcttttcccaaatcccctaattgccaagagagcaatcttaaagtagatgaaaacctaaaggtctctacgcaacatctgaggaacatacgctcctcagataaaagaatcaatctaaatcctcaactgacaaaaaggtccatttaatatttttcattttacaagttaaaagttctagttttgccaccagaatcacgactacccccccttcagaggactccatttaagctcaaaatacgaaatgagcatagggtgaagttgatgtgtaaatggtattctacagattcaagatggcctcttctaaaaacactgaagaaagctttcaccaactctaatttgattttgggttttgttggcagaaaaagcccaagacatctgaaaattactagtaacctccgccatcctccttactaaatgttgtcttctgaatggagttgaaaggtcttccccttagagaggctttccgttttgataccttttgaaagaaaacagcatgcggactcatgttcaattcagtcaccagagccttttagagactattccaaccaggggcaaaaaatgaaccattatttctaaccaaaagaacatggttagcaactctcagctgaatggttttctttttccccagggacatacctaagtatgcctgaaacaacacaggacaatcaataaccatagtggttacaattccaagccattgtactacatgattattgaccagctgccttcctacagatcactgcagactcagacaatggagggctccaaaggaactaatatgctgtgctggcaaaaatagcaagcaccttcctatcccagtcaccacgataggttcacttcatgtccattcttggactagcaggatcaatacagagtaataaggaaaactgtctcaggttaggacaatgaaagtcaccccatgctatatgctccatatttaacactcattctgccaataacacatgtcatggaaatagtccttatagctgggaacatgaaaatcctttgaaaaaggtttttaagtatgatgagcaatcattacaagggatgctttttccacgtaaacaaaagcctggatattttgttaagcgacatttccacatgaagaacacaacaaaaccaaacccatgttagagaatttcttctccctgctaaacacggggacttacaaaaaagggagggttgttcttactctgaatctagccattcctttgcccgaagagtctggggagtaacgttaacatttgatcccaaaaaagtgccgtgcaagagaccacttactggaacacacaattcctgctgctagtactaggagaggtcttatccttacacttcagtttggtcaccagattaggtaagaaagaaaagtgtggggggagggggaggcagaagggtacggagtggggagcgagaaaacagaagaggagaaagaaacaaagggggagaaagagactgattataggagagatcaagaaataagagaaggaaggtgacttgcttgcccaactttggctctgtggtcctatgagccaaaatgcatacttagtgacatgtatctcacaggaaaagggaaaaaaggggtaagctgagagaggtcaagccatggtgttaatttctttcctgtacaaagacagtctcttgaggacaaaggcctgcctcttgcaatgtaatatcatagtccagatgagataatttccttcgaggaaagttggtgagaagttcaaaacgttcatttgggtatcctttagactgcacgtgcttcaccaaagctagcagtttagcttgctctggaagagtgatctgttccctttttccatctggataccgcaacatcagctgtgcttttggtccatttacatctatcccctccactactccatctgctttttcaggtggcatctccagtatctctgaatccacagctggcaatccttggtggtttgtggctgttccaggatcagttctgactggtggctcagtcagcggccttctattctcctcttttctatgccccaaatctttgtggggagactttctggacttggcaagattctctacctcttcttcttcatcagagccacaaacggatatgaactcctcactgccagaaaaaagttcagattcagattcttcatctgagcggctatcctgttttgtctgtgttgaatcaaaatgtgtttcttgtaaggaggctctgatggcagcttctagctggctgtcttcacttgcatctataaggctctctgaacgggcacattttttggggggactgctagaaagtccatccagttgtccatgttcacccagaaatcccgtcacttggtccaagaaagaagatacatctaactggtgccattctactagcttctgacctgtccgtgggtccaatatggaaacataggggaaatcccctaacttataaaactgtatgtatctctgaccttcctcactgtcatgataaacctgccagaaaatgaaatgttcccggataatattcttcacagcttcgttgctccacacatcgcggttgaggcactgacatgcaaagtcttgaacattttgaatgtttatcatcagccacttattttgcatctggccacactctttggctgtttcaaagctgcctttatgcatcaaatcaatgggtggccggaatagatctgcaagggtagttaatttcttatcgatagctcctccatttcttaattcttgttcttgccgaatagtttcagtctgaaaatcccggaaaccatcaaaaattgaacgtgcaggccgtcgtcttttaggagcaccaaataatggttctggttccaccagtatttcctgcttttgaggaattggggcacgaacttcttcttctgtgtgtggtctgacagtagagacacttgctgaactggtactgggctcttcagcgattcctccaccatccaaaaacatagtgactgccatttccagattattgttgcacgcttcaagcatatgttttcctacactttcacttgcaccggtaatggtggtgaactgttgaattaaccccttcagcgccgaggacgccgcggagcccccgtgggcagccatcttaccgccgccgccgccgccgaacaac

SEQ ID NO: 14367 - RNA, 999 nt, Homo sapiens
  source 1..999: mol_type = other RNA
gctgggattacaggcatgagccaccgcgcccggccttgatgacgtctctctttcacttttgttcctgacagtccagactgcacaatttcggatgtgggagactgggtgatttctttgatcttcccaaccaaatatgacttacttaaggattttacatttgttttctctgagtttcttcctcaggaaatggactctcagctctctcaaaaagtatcaaagaagtgaaattcatcagaccacactaggtaaataggtgcttgactgtgatttaacacctgaattactaaaattgattgcaataattatccaaagaaaaacagccaagtgcagcagtaacgacagcctctgaactctctccacatcttcttgtggacagcctttgagctctctccatgtcttctccgggacagcctctgaactctctgcacgtcttcttgcagacagcctctgagctgtttccatgtcttctccgggacagtctctgagtttctgagctctttccacgtcttctccgggacagcctctgaactctctccacgtcttctctgggacatcctctgagctctccacgtcttctctgggacagcctctgagctctttccacgtcttctctgggacagcctctgagctgtctccacgtctcctccaggacagcctctgagctccctccacatcttctctgggtctcctgtggagtctgatcacctttcagttaaggcatctcctgtgagcagcccagttggctactctgagttctgggggtagctgtccttggtttctctgaattgcccagaaaccaacctttctgttgcccatcgtagtgcctacgtggcttagctggagccctaccctgcttttgttgcccaacaaatgcctatgtgacagagctaaattcccattcagctttaactgcttagttttagaaaacaggatgtctggggtcagaagttccttcttaggactaaactggctgaagctggcaaaatccgcaatggcagc

SEQ ID NO: 14368 - RNA, 943 nt, Homo sapiens
  source 1..943: mol_type = other RNA
gctgggattacaggcatgagccaccgcgcccggccttgatgacgtctctctttcacttttgttcctgacagtccagactgcacaatttcggatgtgggagactgggtgatttctttgatcttcccaaccaaatatgacttacttaaggattttaccactaggtaaataggtgcttgactgtgatttaacacctgaattactaaaattgatggcaataattatccaaagaaaaacagccaagtgcagcagtaacgacagcctctgaactctctccacatcttcttgtggacagcctttgagctctctccatgtcttctccgggacagcctctgaactctctgcacgtcttcttgcagacagcgtctgagctgtttccatgtcttctccgggacagtctctgagtttctgagctctttccacgtcttctccgggacagcctctgaactctctccacgtcttctctgggacagcctctgagctctctcttgtttgggacatcctctgagctctccacgtcttctctgggacagcctctgagctctttccacgtcttctccgggacagcctctgagctgtctccacgtctcctccaggacaacctctgagctccctccacatcttctctgggtctcctgtggagtctgatcacctttcagttaaggcatctcctgtgagcagcccagttggctactctgagttctgggggtagctgtccttggtttctctgaattgcccagaaaccaacctttctgttgcccatcgtagtgcctacgtggcttagctggagccctaccctgcttttgttgcccaaccaatgcctatgtgacagagctaaattcccattcagctttaactgcttagttttagaaaacaggatgtctggggtcagaagttccttcttaggactaaactggctgaagctggcaaaatccgcaatggcagc

SEQ ID NO: 14369 - RNA, 915 nt, Homo sapiens
  source 1..915: mol_type = other RNA
gctgggattacaggcatgagccaccgcgcccggccttgatgacgtctctctttcacttttgttcctgacagtccagactgcacaatttcggatgtgggagactgggtgatttctttgatcttcccaaccaaatatgacttacttaaggattttaccactaggtaaataggtgcttgactgtgatttaacacctgaattactaaaattgattgcaataattatccaaagaaaaacagccaagtgcagcagtaacgacagcctctgaactctctccacatcttcttgtggacagcctttgagctctctccatgtcttctccgggacagcctctgaactctctgcacgtcttcttgcagacagcctctgagctgtttccatgtcttctccgggacagtctctgagtttctgagctctttccacgtcttctccgggacagcctctgaactctctccacgtcttctctgggacatcctctgagctctccacgtcttctctgggacagcctctgagctctttccacgtcttctctgggacagcctctgagctgtctccacgtctcctccaggacagcctctgagctccctccacatcttctctgggtctcctgtggagtctgatcacctttcagttaaggcatctcctgtgagcagcccagttggctactctgagttctgggggtagctgtccttggtttctctgaattgcccagaaaccaacctttctgttgcccatcgtagtgcctacgtggcttagctggagccctaccctgcttttgttgcccaacaaatgcctatgtgacagagctaaattcccattcagctttaactgcttagttttagaaaacaggatgtctggggtcagaagttccttcttaggactaaactggctgaagctggcaaaatccgcaatggcagc

SEQ ID NO: 14370 - RNA, 3383 nt, Homo sapiens
  source 1..3383: mol_type = other RNA
gctgggattacaggcatgagccaccgcgcccggccttttctgcctttttctattgtggttctctttccctgagactctgttgttctgtctccaactctgggtgtctgacgctgccctctgggtctctgtccctccctcccccactggctctttttgtttgtttgttgagacgggggctccctctgttgcccaggctggagtgcagtggtgcaatcatggctcaatgcagcctctacctctcagggtcaagggatctttctgcctcagcttcctgagtagctgggatcacaggcatgtgccaccacactcagctaatttttgtattttttgtagagatggggtctcaccatgttgcccaggctggtcttgaactcctggcctcaatcaatcccccttcctcggtctcccagagtgctgagattacaggcatgggccacttcgcccggcttctatcccctgctcttggtctctgtctccccactctggatttctgttcctctcttctgcgtctctgccataccccaccctccaggtcattgtctccctctccctgagtctctgtttctctccctttgggtctctgtctctctgggtttccacctcttcctttttctgggtctctttctctatccttttggctctgtccctctatcatgtctggacagagtacagttttctccccctctcccctttcccttgtggctctgacctccatgtctgagcataaaactgtaggggagaatgggagtgaacagcacaatgaagtggatgtggggtaaacaggaggagcatccacctcttcctaatttacccagtcgcctctggatgaacacccaatcccatggatacagaatccagtcccgccccctacagcgagctggggagccagctcggcacacctcccagagccctcgccactgcatgctcccagatacatgatgcttccccactgctatttcctttgggtcctggtgctaccactaaatgcaaaacagcccgatgtggccctatggaactcgttcgcacagtccaactcaacccaacttcctgtaggactcacatagtgacacaactcaatggaactcaattcagcatggccctatgagactcaaacagtggcatgacccaactgaactggccttacaaggctcatatggttgtacaattcaacacaactcaactcgctgtggccacgaaaaatgtccagccacacacctctacacagttaagcccaacagaaccctacaagattcatttggtcatacaaacttaacccaatgtgacctagaaagctcaaattctaccactggactcttcacatttctacatgactcgcaagttcacagaacctaaaataacatgcccctggaagaatcacagagctacacaatttccaccatgtctcaacgaaacttaacaccacacacattcgatctcaacaatgccatgggggaccatctaacttgacccaacatggccctaggggacccaccaaaccacagaatcctacacaatgcagctggaccacactatcccagactcacaacccaaccaaacccaacactgacctaggaaactcacaaaatgatacgaccaaacctatctcaacactaccccaaaaggctccatgagctttgcacaactcagagtaatatgaaccaattgagtcttcattaacacaacacaacccattgccattcgctgctgcttcaggaggtacccacaggagctaccaaaccacacaacccaagacccaacaagactcagtgtttccccactcgttacgacttaacctagctcttcctaaacccaatcccctccccccagccttgccctccaccctgccctccctccctccctctagggaggtgtgaggtcctgcagacctcaactgttcctcacacttcggtgaccaggtgtttccctgggggtgcccagagtggaggtggtagctcaggtacctccccgtccaccagccccccattggccttgccctccagtgggccacaaggctgcatgtccacatggctgaacatcccagcctcttcgccctctgtctcccggtgataaaagtagctgaaattggagacaatgacgggcactggcagggaaatagtcagcacgcccgcaatggcacacagagagcccactatcttgccacccacagtgacgggtgccatgtctccatagccaactgtagtcatggtgactaccgcccaccagaaggactcagggatgctagtgaaatgggagtccacccggtcaacttcggcaaagtagacggcgctggaaaagaggaccacaccgatgaagaggaaaaagatgaggaggcccagctcacgcatggaggcccgaagcgtctggcccaagatttgcaggccctttgagtgccgggacagcttgaagatgcggaagacacgcaccaatcggatgactctcaggatggccagtgacatggcctgctggcccacccctcgctgccgggccagctcggtgcccagtgccacaaagtagggaaggatagccacaaaatcgatgaggttcatcacgttcttgaagaagatagccttgcttggacagaccaggaggcgtaccagcagctcaaaggagaaccaacaaatacacagcgtctccaccacgaagaacgggtcattgaagggcaggcggggtggatttccaggcatttggctggagccattcagcggagcggggaacgggccggctgcggctgcagcagcaagccccgtgccgtcgcggtcgtcgcggaagtcaggcagcgtctcgaggcagaagacgacgatggagacgaggatgaccagcacggagactacggcgagcacgcgcgcggcctgagagctctcgggaaactcgaaaagcagccacagctggcgggcgaaggcgcggcggggcagggggcgctcgggcggcaccgggcagccctcgtcctcgcgcaggcgtgccagggccgccgcgcccagcccgtagaaggccacctcttccaggaagacgtcgagcggcacgtgcgccggccgccgcagccgcccaccggactggtagtagtagagcacggcgtcgaagctgggccggtgccggtcgaagaaatactcgcggcgcgcgtcgtcgtagaagcggccgcggcgcgctgggtcccctagcagagtgtccgggaagcggcccagcgtgcgcgcccgcgtctcgaagcgcagcccggccacgttgagcaccagccgctcgcagcagccgcacggcggcgggcaccgcggctccatggcgcgcgcagccccggcgacccgcgaaccgacgtgtggccccgacgcccggccccggtgcggccccgcctcggccgcctcggccgccgccgccgccgccccagcccggtgtcc

SEQ ID NO: 14371 - RNA, 1219 nt, Homo sapiens
  source 1..1219: mol_type = other RNA
gctgggattacaggcatgagccaccgcgcccggcctttttcttctctttttttatagcagcaggtcttatctgtttttcccacaaaatgctcttttgtgagtattccagggttggatgcaattctggtatgttactctaatgctacttctcccactgacattcaagaaagcatcagaatgtgagtgagtaagggtgtcattattatagggattaccttgaattagttctattttatgtttattttaaaaaacaaggaaaattcctcctaaacctcgatccttaatgttgcttatggcaattgtctgtacttcataattggtagttctgtaccagtgccatggcttagtggttgagagctgttgctctgtaaaacttcgatcacaacttgagttggtcaccatttcacctgaaatttattcctttctaagctccttcctttcaaccatttttcgaatgcttaccttgtgtgaggtagagggccaagtgctatagatatatgtaaggtcacattcacaggtaccaggtgcgaggactttagcatatttttcttcaggacacaattcaacccataagaagtagtaagtagattatgatgcagttatgtaattcaccttgtctcacatgacaaggctgttggtagactcagcaactgctttttttcagtgtatagctgggaacccaggaagatgttagaagattatgtaaatcagcttttctgtattttaattctcctgtgtcttcatagttggaccagctaataattcttactttgaggaaagagctctatttaatggctgtactgatccctctgtgggaaccttgtagaagctgcagagaatctgtcacctttcttgagttagtggtcttttcattttggggtggttccgagggtctcagataacagttattttcctggagaacattacgttcagtgaaataagccaggcacagaaagacacatactttgtgatctcacttatatatggaatctaaaaaaatggaacccacgagtagggagtagaatggcagttacggcggttggggggaacaggggggtgtcagggagatgttggtcaaagggtacaaaatttctgttaggaggaatagaggaataagttcaccagatctattgcacaacatggtgattatagtaaataacaatgtactatgttcttgaaaattacggagaggttttgtgttctcaccacaaaagaagta

SEQ ID NO: 14372 - RNA, 1160 nt, Homo sapiens
  source 1..1160: mol_type = other RNA
gctgggattacaggcatgagccaccgcgcccggcgacttttttttttttttttttttttttttttttttttttttactcccaagcttcccagttggattgtaaatatgtaatttgtgatatattgacaaaaaaacacatcatatatttagactttaaaatgacaccaaaacggatagggctataattaggcaataaaaagaaataaaaggtacaggctgggcgtggtagcttatgcctgtgatcttaatactttgggaggctgaggcaggagggttgagtgagcccaggagtttgaggctgcagtgaactccagcctgggtgacggagcaagaccccatctctaaaaataataaaaaaataaaaaaaaattaaaataaaggaaataaaaagtgcatgttgtggaggtgctcgcctatagtctcagctacttgggaggctgaggtagaaggctccttcgagcctaggagtttaagaccagcctgggcaacacagtgacaactaatctcagaggcttgattcattttagctgcaaagaaaaccagtcctcgtctacctttttcgcgtgttggagaactaactagcaaggcagggaatgcggttcgtgggcgcttggcctcctcaagcggctcaggctctcagagcgcgaggcccaggggctctggagccgcggccgcgacgcgcccgagggccgttctcttcgacggcagagcaagagtcaccgcgcgggagccccgagcgaccgccccgctgccccggtaccctcccctcgcagccgcccagagctcttcatgccccgtgacgcccgttagggcagcgcggccggaggccgggccggacgtggcccgagatgtccgggggcaggcagaagaccacgggcacgcgacaggcaaccgccgcctcggctctagaggtggacgttttgtctccctgcgcttcaataccagattttgtttccagacgacatccctgttgcttccggcacttggaaagaccaatcgtcaggcccgagaatgcaagacccaccctcctttgcgacggaggcagccaatccagttgctcgctacttccagtgtcgcatgcgcccttacgcaggaccctgcccaatcgttaccgggacgtcctcctagtcccgcctccggaccgccagagaggctgtcaa

SEQ ID NO: 14373 - RNA, 2902 nt, Homo sapiens
  source 1..2902: mol_type = other RNA
gctgggattacaggcatgagccaccgcgcccggcggaacttttgcaattttcaaacatgtttttttccaagtaaaccaatcaattcgaactcaaggttccatatcatcattagcttgatctgaaagattaagaactagttcttacatcattttctgcaggccatgaccttaaacgcctactagaatggctataatcacaacagaaaacaatgatgacccatttccaatctatagtcctggatcaaatgcaactgagcaattctggcccagaaattatacttcacagacaatgcaatgaaacgcagccaggataaatgctggaattgccccactctgagtgtgatctcactaaagccctcaactatctttccacaaagccctggggagaggcagggtcaatattgcacatctgtcttcaaggatgaagacacagccccttaactggcagggcccatcactctggctgaacagagctcaagactgtttgtccactggctattcattccctgggtccctgctctgcccatcctgtggctctgtggaaagtggcagctgtccctgactcgctgctaagctattgctcagtctggctccacagatgggaaacacacaaatgggaacaccacagaggtggagaggtggagggtaggtgtggggagcatcagaagatgcaatagggagggaaaagccctgtgggctttgagtatcccacaaggatggcagtgcctctaccgtttcagggctcctgatagttactgaaagggctgggagtccttcctgtcactctagtagattcaacaaagggaaaacagccaccctactgattcctatccaaaagcagtgattttctcagttgcctccagagtggtttttttttccctcccagtccttggcttgtcttgctgcagggtaatctgacacttttcctcaactgtggcaataagtgaaaggagagagaacaaaagcatctgaatcacaatttaggcaaaaagctgacagccacacaggctgttaatgagggactctctctgtctcaggcagcgtatctcaggacacaggtgctgagaataagagacaggtagcccctgtgttagtgaggcctggcaccaatcatagcacatcctacgagacgaagaaagcaggacaacactctgcctagttattagggtcttttcgggacaggaggccaaactgggcagctcctttacaaagtctggagacattttgtacagaacaaggaggaactaagtccacttcactgcaaagtgacctgagaacaccctctagtggaaattattaataaaacaaagaccatgcgcctaattcaccttctgatacaagaatggtttttaaattccccataaaatggaaaaaacaaaaaacagaaaaacaacatattatctttaagaacacaaaaacaatttttataaggcaggagttcccacccatgcttagtaccctgactgccaaatcacattccttcctcagagactctgactttaatatattctaagaaagggagacatgtcgtggggggagctacttgtccccttaaattttgggcagactgcctgctggtgccagaatgatgccaaagacatagaaaagtcccagcaggaggttgagcttggcagtcctctggggcagtttgttgaaggcctggcttcgaaactgtctctcaagggagaaggccatgggaatggtaagcagggggagtgccaggctgatggtgcagtgtgtggccaggatgctgaagaccaggtagggcaggaagagcagtgtgttgtagagaatgtaggagaacgtggggccgatgaggatggccagcgtgacgataccagcctcccggtcggactccatgtccctggtgttgttggaatggagaatggcctcggtgctgagggcgagggggatggcatagaccagtgggaagatggccagggaccccacctggatggcgtaggcgaacatcacagccagcgggccaaaagtgatgaggatgatgaggtctcccagagccacgtacttgaatccaattcctcctgtgtagagaaaggagccagacaggcctccaaagtagataagagccaagtgctccagtttcagaggggacaggtagtagaggcaagcggcacagacgcagcccaacgtgtagaggaagactccgaaccggacgacatcctgcggctccaagattcggtccacaagtgtcctgtcatcactctttttgtggtcaatgcccttggaaaagtcatagtaagtgttgaccaaattaccggccccgtgcacagccaggacagccacggcacaacccaccaagagcctgggatccaggacaccgtgggatctgtaggcaagggcactgcccagggccaccggtgtgagtgaggcactgaagctccagggcctcagggccaacacgtaggaggcacacttctgcctccaggagcgctgggggagcctatcttgctcgggacagtcgttccccagcgggtccctgtccccagctttgacagtctctcccgacaggatgttaatcttctcccccaggacctgagaggccgccatggaagctccacgtggttgaagtaaactctaaaagtgagccacgcacagtgaccgcccgggaaggaggaaggacggggcggggcagcagggcccgaccttccttcggttccgccccaggacagggctggtgtggcggcaaggtccgggggcaacagcaagtgggtcttacaccccacgaggccaagcggcgccgcccctactacccgtcacctgggcgaagtctgtctccggcccccagccccgcgttagagcccacggctgagccgcggccgccttctttaggccgccagagccgccatcttgtgcgccggcctctggaggcccgcccggaaac

SEQ ID NO: 14374 - RNA, 3319 nt, Homo sapiens
  source 1..3319: mol_type = other RNA
gctgggattacaggcatgagccaccgcgcccggctcaatattttgttttttaatgtgagggcacctcatgttatcaagacatttgctatctgatcattttggggggagtggaaagaacaggcaagaaaaggaaagcaaagagaaaaggagaagggtagaaaaatccttaaaaatattttggtgaggaaaatgtttactgagtgtctatttacaacgaggcaatttacacaatgaggattcaaaagaatatgttgtatcaagactctctttgccaggcatggtggctcacgcctgtcatctcagcactttgggagacctaggtgggatgatcacttgaggtcaggagttcgattgagaccagcctgtgcaacatggtgaaaccccgtctctactaaaaatacaaaaattagctgggcatggtggtgggtgcctgtaatcccagctacttgggaggctgaggcaggagaatcgcttgaacctgggaggtggaggctgcagtgagtggagatcgcaccactacactctagcctggattacagagcaagactctgactcaaaaaaaaaaaaaaaaagaactctcaaaatattctaacattctaagtccaaaaagaaagatataatagaactatttatttgtctatgcattaaacttctggtaatttcagctatgttatacccagttataaattaaaaagagatcaaaataaaactcagagcctatttccttttcctttatatagaaatctttcaagctcggtgactaggcttttgaactaatgtaaacttcgtgaggcttcatgagaccatttctttcatagccccagtacttaactcaaaacctagtttatggaatggattcaataaatatttgttaatgaagccaagtgattagataaacaaaatggagtataaccatgcaacagaatactatcaggccataaaaagaaatgaagtgctgatacattctacacatggataaaacttgaaaccattatactaagtgaaatacgtcacagtaggccacatattgtataattctatttatatgaaatgttcagagtaatgaaaatccttagagacagaaagtaaattaataactggcatggacgggagagcagggagcgactgctaagagtataagatttctttggtgggtgatgaaaattttttgagtgtggtgatggttgcacagctctgtgaatatacaaaaaatcactgaattgtacacaatacaaagttgaattttaagttatgtaaattttgtgtcaataaagcagttattttatacaagataaaaaaataaagatttgttaatgaatgaggagattagaagcagtattcagtagctggggttgttggagaccggtacacaaaattaggagacctgatggctgacaccctggagtccaaagaaagagtgagaaaaatcataaacccagacacaaaggaagaaacagtcccctacatactttactgactctaagggattatagcacagatacaaaaacaattggcattaacaataaagaccctgagtcattaagaaaatattgatctttgtttaatatacatcatttaataaaacgcagggagggagctgtacaatgcagttttaagatatttttattggactggattaaaacatcactctgagaacacttagtcccctcacatgctagatttccttttcaaaatgtaatcttgatgatataataatgcataacttaaacttcccttcccttcaaaacatccttggttctactcaaggacctctaattccatagtatcttttgtagacacagaaagtatgcgttttctttgtctttgtgatgtattacacctcccagtgcagaattttaatatattccacatatcatatcttcctgtttcggttacaaaacagtacagaattggatcagcaacacaatttaaacttgttaatgcaaccgtgattctatacattgtgtaagttcgcttcccagaattgctgtggtcttcgaagttcacagcatgctctaaaatgcagcgaatcagcaacatcacatgaaagggagtaaagcataagacaaaagtaactgtgatgctgacaagtagttttatgattctcttcttttccttgttttccgtggctttattgtgccgcacagcttggtagactttccggttgcagatcaggatggtgaccaaaggtattgcatagcctgtacacgtcctgaacaagttgaggttgatttgccatttctctaaagggtatttgtcatagcataaagtaaaattagacttttcggcatcgcaatattcaacaactgtttcatcttcccacaacatgacagcattgaagatggtttccaatatccagatggacaggctgaccatgagtgcaaatcttcttgtccttaggaaaaaaaacttcaaagggtagacaacagccaaataccgatcaacggcaatgcaggtgaggaatgctgtgctgctgtaaaaattcatgtacatgagaaaagcactccctttgcacaaggcaggagagaaagtccagttgtctttattccaggtataatcaatccataaagggagagttaatgcatagagtaaatctgatagtgacaaactgaagaggtaaattcctagttcactttccttctttgcttgcaggaaagacacacacagagatccaatattggctggaatgctgactataatcacaaagatgtaaacaatgggaaacaaatagtgatccaggtcatgctgttcttcaatacatgtgctgttcattttttcctttttaaggtagcaattatattagttcttagaaagtaaacagagaagtcttgtctctttgtagtttgttttgaacatcgaattcgcttttactgagaattctttttcaatttttctttgttgtctaaagttctaattaattcatcaatgcttttaaagggtggatgtagatcaatttttacacagatatcagcagttggaagtaaaaatccaggctcctggcaattggctaaaggggtcaactgaatttaataaacagaagtccatgtgttcattatcacagaacgctgacaaacagcccacaagcatcaactgaggcatttgtaagtgtacatagagagttgtccgcaatttgtttttcttcataaatctcacagtagattggtgcaaacatgaatatacaaggctttgtttgcacagagattggtatttccttttaaaattcctttccttccatatttcttccggtgatgtgtttgttgactgaggagcttgataaatctgtgcctgcatcaagtcaagaagagaaaccaacactgct

SEQ ID NO: 14375 - RNA, 955 nt, Homo sapiens
  source 1..955: mol_type = other RNA
gctgggattacaggcatgagccaccgcgcccggctgaataatttctattgcaaataaataataaagtatttctgccttttgaaaattttcctttgttagtcttacagtttcagagagattacatgaatgtctggtaacttacttattattgcttttcctttggggagtgataaaagattccggagttatttttgaatcctggggctctgaactcatgtgatccttacttccaaataactttaagcaattgaaacttaaaagcacactgactttgtattatcacagttttactttcacagatgtctggctattcaattcatttagtatcatatttaagactaccgtaactaaatgtaatgctcttagactgtaagaccattgaggacagattctataacaaagtagattgtgttactattcaccaaatattcgggtttctctccccgtggtgccctcccccgtaagagattatgtgtccccttttggctgaatttaggaatagtcatgggaggaagtgacatgtaagtagttctgtgcagaagctttgagattagtgcttgattcaccatttctcttttctctcaatatcccatcaatatcccacgtcaaggctcctcaatcgaactgggtgtgctagtgaagatgatgatggagtagatcctgcgttgacctgtgagagacccttcggcttccagggccagaggtcttgcattggctctgctttgctctctgttctcctggccatcctcagacccagagccacaggtaaggtaggctgcttcttagcctttctcttttctccagcagactcggggcccaaattgggaccacacatttctgccatcgcagacggtgggcaaacagctgtctccacagctgagaccactggagctgcttgcgctgctccagtaactcgagagcacacggctggtccctggatggcacagagcactgt

SEQ ID NO: 14376 - RNA, 3557 nt, Homo sapiens
  source 1..3557: mol_type = other RNA
gctgggattacaggcatgagccaccgcgcccggctgatatatatattcttttaaaatctatacacaaggctcaagttctggggtttcaggttttatttttaagttttctttaaaaataaaattgccaacccccaagtgaattaaaggttgatctgggctcgcagaggtaatctgctctttgtaaccaagtgctctgtagtttcttccactttagacctctccagtgtgttaatgcctctgttttctttgtcttttccatgtgattttttatgctggaaaaatggaaccccgccaattgatgaacaatccacaccagcatctacagatggctcttgacttagaggttcttcagtatactgccccagaactgcctcttctacatccacatccggaattgtctcttctttgttgttttctgaacagtttagcatcattaacagctcaggctgtttccttttcagctgatcaaggagatgttcacgtggttcagttcttaccagtgttgatgggtataaataacttttcctctgtggtgtcgtacctgttgggatatccagtttcagatcctgttccagaaagcaattaagcttagtcaaaccaatttttatggtttcattaagttctagattttgtgctatcaatttatcttcatcaatagtcatctgatcaagaaaaatgttatgctgtttctcatgagctgccttacgtccatctgatttctcagtgatgtctgaacttgaagcctcacaacattggcttacaacctccaataagttgtgaagttcctgttccctttcatttaaggaagatacccactgttcagaaaaataaactgttcttgtgttcagagattcacatctctgttcagtctcttgagatattttttccaggttgccattgagtttatcagagtgtttcacagattcttcaaccaattttgtaccttcttggttaaaatttctgagttcctgtgagaagccatcagaatcagcacaaaatttttgactgtgaaaagtcattttgttgactatatccttagatttctgctgtatattttcctggacactactaagtggtttctgtatattttcacacttttcctccaaagcacagaatctctctgtccaaagattcattaacttgcaaagttcctgggaatgggtctgctttattgtcttcaggtcttcagttaggtttccacattgcttttgtgactcaaccaaggaacaaatggtattttcttgtagttcatgtagattgttacacagtatactgagaaagccatctagttcctttttttgatcttctatcttatcggccactgtcaatgaagtcttgaaaatatgctttagttgactattgattttcagtatagacaccacagttggggataaaatcatttccagtgaacttagaagatcagtcttgagtacattaatcaattcctgtagtacagttttactttctgctgctaatgattgttcttttagtatcatattaaaaatctgagaaacatgagtagacacattttctggaatagatgtgagagatccaagtgctactgtagtaatggtatctaatgcagagacactggaagacagcagattaccaaataaggtcttatgtacttctagcatggccttttgctttgagctgccatccttaattaattcttccatattattaaacagactattcaggtttttgccaaaaatatcctgagcttctgcattgtgttggtcaactgccttcttacgatccagtttggaatggagaccagatacatcttttgtagtttcttcaactgtgttaagcagcttgctggcagcatcatgaagtttctcctcagtactttccaaagctgatgtgatatattcttctttaacaagttgtaatttagtttcttgcaaatgtttttgagtggtttcaagttcttgtgttttattttgcaggtcagatttacactggtcaagttcatttttattatccataaacaactctgtaaccctattcagctcctcctcaacagcaccaattttttcaatcaattctacaatctgctcttcttgaacagttaattttccactcatgactctaaaattttcttcagaaatatacactccatttttctcacgggctgcagcaagatctcgttttaaacgttctatctcctccgtatactccttaataagagcttttttggtgagtttctgattcacttcaggcttattcaatatgttctttgctctatgagcatattccaatgtactcagagtttcctcaagattgagagatgcaggagaaattgttgcaattatagatgttcttgtacgccctccaagagaatcctggaggattctagttagtttagattctcgataaggaacatgaggtgttctttctacaagggcagtaatgacccttcccaaagtcaacagggattgatttatatttccagcttcccgagctctcttatcaacagctccagaacggccaatgttttcacttcctgcaagatcaaccaagttcaactttccgattttaacaagctcttctccatcaatcgtagtttctttcatatgtattgtaacagagaaaactgagtgggaacgactagagtatgcattcatcagagtagctgcagttgtcctttttgctgcccccttttctaaaatttgatagacttcatccttgttgtgtactgtaatttcttctaaacctttaattatcactcctctcttgttacggggatcatcaaacatctgtagtctctcagaaacatcagatgatggattaagaagatcaaaaagctcttcattatagatctccaacagagacactttgactgaaaattcagtaccattatcagtaagtttctcaaaaatttgatgaagggtacgtggaattataccagccaagggatcctcttcccaggtatactcttcattaggtgacctttcaccttccattgtaaaagtttttccagtgccagtttggccatacgcaaagatagtgcaattatagcccataataacttcatccagaattggacaaacaacacttcggtaaacatcaatctgtttagtagatgctccaaacaccatatcaaaagtgtatgttttccttgagctcttgtcagccaatcctccagttcgtacactaacttcttttcgtacaggatcacattctactattgaatgggcgctagctttccgctctgccaaattaaatggtctgcatctcaccaccacctggatgttcttccccttctcctctttcttcttcgcagacgaatttggctgcgacgccatgacggtccccgccaaaaaatcaaggcccggccgcggacctgggcgctgtgaggggcggaggggcttggcggccgacaggggccggagtctccctggtccctctcgggcgctggcgtggcctggaggaccgacgcacgcaggtcggcgtccccgctctctacccggtactctggccgtggcgtttgtcccgcgccagtcggagccgccaaatcactaatctcgtctccgcccgaatccccagaaact

SEQ ID NO: 14377 - RNA, 1620 nt, Homo sapiens
  source 1..1620: mol_type = other RNA
gctgggattacaggcatgagccaccgcgcccggctggatcgtatctaattttataattttaactttttattcttttcttgaagagggccgctgtggtggacactataagcaccccctcccaaagatgtccatgttttaatccttgaaacctgtgaatatgttatgtaatatgacaaaggataattaaggtgacagatagaattaatgttgctaatcagctggccttaaaatagggagattatcctggattgtctgggtgaaccgagtataatcaagagtccttaaaatggaagaaggtgacagagaggaggtcagagtgaagcaatctaagaaggacttatctgttgttgctggttttgaagatggaggaagaagccacaactcaaggaatgcagatggtctctaaagctggaaaagacaaggaaactgattttttcccagagcctccagaagggaacacagccctcttgacgcttgagttttatttagcccagtgagtcctgtctggaccttttaactacagagctgtaagagaaatttgtgttgtctaaagctacaaagtttgtggtaatttgttatagcagtgatagaaaactaatacagccaccttagatgtgcatacttcaggccccgcaaaacttttatcttccgctgacagggaatataaagagtacaggctttgaagttggaaaacctggtctcgtaacttacttgctgtgttactgtaggcaaatcgctgaactcttccaggccttagtttcttcacaggtacattggagataatacctacaaacctgatctgcttcccttgtcttctgctcttctcctctcctggcgagttggtgttggttgttgtcaggaagcctcagctcctcacaatgggaactccccagagggctccttgaatgtcctcatgacatggcgcctaactcccaccagaatgagagatccaggagacagtgagagggaagccaccaagcctttaggtcctaatctctaaagtcacttcccggacttgagggacctgtgactctaggcaattgagggtagttgtcttgccaaggtgatagcatgtaatagcccataattacccataatgacttcatgaggctcagcctaggtgggagcccaggcatttcaagataatgtcttttcttccctttgtattctgagtgtgttagctccctgcatggattgaaaggtgcttattaacacaagtgcccttgttaattaggttggttctgacttacgtgctacttattagatactcaagtcaatatggataagtgtcctgcttctgggccagggacagagaaaaagccagaaaacccacttctcctcaaaaggtgtctctggtgtccagaaaggacagaggatgcttcatttttatggtgctgggatgagctgagggaaggggagaagcaggaggcaaaccctggtgggggcgctgctggaaggagacagctcacaggacaccaccaccacaagctgagcctccactttcccatctgtgatgtggggtttagaaccagagtattggcatgagaaaggattagagatgaatgcccacttttgtccttgtaagaaaaaattgtggaactttgaaattaagtaggagtc

SEQ ID NO: 14378 - RNA, 559 nt, Homo sapiens
  source 1..559: mol_type = other RNA
gctgggattacaggcatgagccaccgcgccctgctatgttacttatttcttaaacaccttttatgcttctttctctgatctgtgtcttttttctttgacagcatctccattttttttctgctgcttcatcgctgtagccatgggaatccgtttcattattatggtaacaatatggagtgctgtattcctaaagaaactgacacaggagaatcacttgaacttgggaggcagagtttgcagtgagccgagattgaaccagtgcactccagccttggcagcggagcaagattctgtcacagttcctgaagtgctggtatcgtcctgcagccccatcctcggttccattgcgctgccaggcagggtgctgggacgtggggagagctggtctatatatccgggtgaagctcagctgtggcacaccttggatgccgggtctctcctggccccggggacctagtatcgcaggcaaaggggacagtaaatctgtcatctccaatcctgatgagcccccagaaatgtatcgggatatataaggaatcagagagaccaagggattgag

SEQ ID NO: 14379 - RNA, 1091 nt, Homo sapiens
  source 1..1091: mol_type = other RNA
gctgggattacaggcatgagccaccgcgccgggcagcttacagattcttgcaatagtacttaaccacacgccctcctagccccaaagtaacgaatcacagatatttttaaaaaagaatcaaagcactctggtccaaggcagaccagagttaagtaagcatctggtaggtgtcatagtccagcaatactgtaagtttatgggaaagggcctatggaaaccaatgactgtatatagttcaagttaagtggttcaaaaatttcgttcattattctctgccatgtacacaagcctcagaccctctaattccaaggaaaattatccttggcctctgaattctgtgaattgtgtacattaagggagatctgtccttggcaagcagaacacgttgttggcaagctgcaaataccttccacccttttgccaaagtcccctcacagggcaggctcaattcctcaaccttcagacccaaaacggcttggtattacacaacaatccaacaagaaagcaaataagtatgtacgttggaagagattacaccacttttatagttactgggctggagccactcatttttcagcggagagggttagaactgggtaatgaaggtaaatcccgaggagtccaggaatagcagattcactgattcactgactctctgggactcgggctgccaaaaataaaatcccagtactgggggctccgatcagtcttggtgaccagcactaggcagcttcaacctcgggtgcctgaaagtgctgggtgtccagtggcataagtcttctttgatacccagtcctctacaccaacaaagccgaggtccggaatgacagtccccagagaagcggagtcacccttctcccatccggctaggccacaggaacccaacaaagttcagtcatctggtgcaccagctgctggaagcgctgcttttgagtctctacctcgatgaaatgctgcaactgcgggtccactgcacccaaacccgccgcggaggaagaggaggaggaatccatcccagggcgaccaagcttgcagagacgaactccgcaccgaccttcacgtgtctccgcgacggaaccggaaccacagct

SEQ ID NO: 14380 - RNA, 1107 nt, Homo sapiens
  source 1..1107: mol_type = other RNA
gctgggattacaggcatgagccaccgcgccgggccggaattattgttctttgctctcaattctgtatgacatctaagctccaaaaggaagaaggagaggctgggtaccctgtgccctgagctcagaacttcagggggatgaccggccagtacttgggctgctttcggtcacagtgcttgtcaaagctcagctgcaccgcggcctccatggcttggatcttggcagcactgtccccgtacaaacgcttcatctcggcctggcgccgctcaccaggcctctcagttggggcttctaccgaccggcgggtgttgcagtacaggtcgtggtcagcgttcacatagctgtccaggcgctctgcatccagctgctgctgccgccgtcgttcttctctatgcctctcggtctctgcaaagtactggcggagctcttcagtgatttccatattgctcaggtcacattctacctctgcatctgactcagtctccatctcttcctctttggacaaagcttggtcttcttttgtggatgcctggatcctactgctgtaacgtggatgctgcccagatcttctgaaatgtgaagaactgcaggggtagtcctgccaggccacatgatggtcatagaaggactgaggatacgcagcctcattatcgtaagagctttggggaagaagcgcagaaggtaagtaccatggaagattgaaacaggattccacggccttcctgtaggcattgtgatggctttgcatccaagccattgcttgatgataatgttgccagtatcttgcatataccggatgagaataccaaggcctggtagctttcgatgttgatgcctttaccgctgccatctctgattgtgaaagtccaaatgggtgctgaaactccctgggaatgtctcccactcttttatggcacaagccttcagggactgaacagtaacttttctccaatgggctggtggagctcgtgggcgcgcagcttgcggatcctgggcgttggccgcgcaggggcctagttttccttggagagacagagggggagtgggggacgcgagggaggcggctgttgccggggcgactggaagcgcgcttccggtgcggaacac

SEQ ID NO: 14381 - RNA, 4661 nt, Homo sapiens
  source 1..4661: mol_type = other RNA
gctgggattacaggcatgagccaccgcgccgggccggaattattgttctttgctctcaattctgtatgacatctaagctccaaaaggaagaaggagaggctgggtaccctgtgccctgagctcagaacttcagggggatgaccggccagtacttgggctgctttcggtcacagtgcttgtcaaagctcagctgcaccgcggcctccatggcttggatcttggcagcactgtccccgtacaaacgcttcatctcggcctggcgccgctcaccaggcctctcagttggggcttctaccgaccggcgggtgttgcagtacaggtcgtggtcagcgttcacatagctgtccaggcgctctgcatccagctgctgctgccgccgtcgttcttctctatgcctctcggtctctgcaaagtactggcggagctcttcagtgatttccatattgctcaggtcacattctacctctgcatctgactcagtctccatctcttcctctttggacaaagcttggtcttcttttgtggatgcctggatcctactgctgtaacgtggatgctgcccagatcttctgaaatgtgaagaactgcaggggtagtcctgccaggccacatgatggtcatagaaggactgaggatacgcagcctcattatcgtaagagctttggggaagaagcgcagaaggtaagtaccatggaagattgaaacaggattccacggccttcctgtaggcattgtgatggctttgcatccaagccattgcttgatgataatgttgccagtatcttgcatataccggatgagaataccaaggcctggtagctttcgatgttgatgcctttaccgctgccatctctgattgtgaaagtccaaatgggtgctgaaactccctgggaatgtctcccactcttttatggcacaagccttcagggactgaacagtaacttttctccaatgggctggtggagctgaaagaaaagagattggcaatgtcagggaaggccgggatccgcagctctacaaacccggcagccctctccagtgagcacaatggcataatggccaccacccagctgagcccaggcgagtacagagaccattcattgtctgtcctcaaccaccaaagaaggaaggaaaaaaacagggttgaggtcattcactaaacactgacgaggcctataggcaaggcagagactgagtcttgaatgatatatttttccatatagcctctcttaaaaaacggatttacacttcagtacatctgctcatcctgcaggatctatttttaatgcataaatatacacaaagaacaatagataagagctttgtagttttcaatggataaaatgtgactatttccatcaagttaccaaaaaatttcacaaataagtggctttgttgacaggtagtgccatcaaatatattcttttaattacatatttatgttcttataaatatagaatataggacaaatcgtagcaaccaaaaaagtaaaataaaaacacaaattcccctaaaaactagaatgtatacttgaactagattttcctatcttccttttctactagaattctaaaaatacatgaaaattcacctgctttgatctttgcacagaaacacattaaaagccaatcattaaataagttactctggctaaagccctgaaagtcaaaccttccctacaaagctccagtgatttggttctctgaaccaaccaggtaatttggaggatttagttaggtcttcagtacacactgtttcaaggagatctgctggacactgcagcaaaataagtgaaggtatggtgagaaatctgagtgagatagattgagtcatatgcggttccaaggaatctctctgtacatgcaataataaccctatcacagaagatgtcttccaataatacacacaacagtaagaacttcctcactaagacaaagaatataatagggttttgttgagggctgggcttcctgccccacctacttgggcagccctgcccccatccctggctggttgctgaggctggcaagctcatctggcttgatgccctcatggcctccctcctgtgtctttgcatggtccctgcttagtgatttggacatcaaagatggctcaagtccaaatggccttcttccacctgcagacatccaagctccatcttgggcaggacacaggcctactcaagtgcacatgccactgtgttcagaaagcctgcatctccccgtctataatagctacagttaaaactgataggcaagggagccaaaaaactgagttttattttcttttcattccctcaatccccaaccccaatttaccctcttctggatgttgtaataagtactgtcacaaagaaggcatagcatggggaaggagtaaggctgaaaggatgcagttaacaattctttttttcatacaaatgacattccacccacagaagggcattgtttaatttgtcagcaagtgtgatgaatttgtgaatgggtttatttgcaagttctctgaatccccttgtgactaatatcagaatcaaaagtgaaatatgaggccaggaacaaagttaccctctgactcaggaacacaacaagcaatgggatgactgagaatgacataatgataacatagttcaaaagaggaaacagataagtttgtttcacagcaagcatgtccttcataagcaaaacctagtgtgaccataaggtaataagggttgaataggcaggttctgcaaattaagagcataacagcaaaaaccatggctagtttaaagtagttaagatcgctagtacatttcaggcgtcttatttcaaatttacttttttctataaacatattcacggtaattccatgttaatctctcttttctgaatttataggcactcactatgcctcatttacttgggcacttactcagttacctgtaggcatggattctacaatctactccttttaagtttcctattttccttccagcataaaaataatagctaatatttcatgctcttagatgctgctgaaattgttgagcttgtctgttgtttcctgataacgttctctcctcctgcatctactccccaaaatctctgaggacctagtaactcaaaaaactgactataaagcaccaaatcttttcaggaagcaaatatttaaatacattatgttttcaaagatcttttcaattcatctgatatttgatcaactacattcttttttcacttgtccagctgttccgtggctgaatttcctcttgtagagaagttgttcaaaaaaagttctgtacctactttgcaaactctccaatttacactctagccttaactgttcaaaactttcccccgtcattctcatctcaccctatcctttaaaaaaaaacccaaaatgattaatcaccatctatagaacagtttcagaatgaacatttctctctggaactttagtttgtatacttccccagcacagcaatgaacacacagaggggatttatacacctgtgaacttgctttcagttatgcttattccaagttactaaccagcagtctttaaaaatatatggtttctgttcacattgaaattacaaagagactgttattccgataaattatgctagcaaaaatagtatttttaaagggtagctctcatcctacaattcatgggggctgtgagcataaataatcctagaagtgttgcgttactaatctttagtctagattttttaagtaatattgttctgatttgagatgaagaacagctgaatacacagcctagcctgtcaaacgagtttaaaaacatcattcctgaaaaaaataaaattgttcagaaccatctgatctgtactaagggaacatcaagatttcagagctaaaatgcacttcgttggccactggttcaattacagctcattactgataagtgggcagagacacaaggcccataaactgtaggcgccagatgtctcaagataactcccaccaaaagctgacctcctgcagaggttaaagtgcaagagaaaagaaagaaacccgaatttttgagcagagagggcaatatcctagacatccttcaagtatgtggctgtcctgggcgatcttctattcagatactggactggatgggcaaaatccgaattcacctacagaccttaacacggtggttctcggcaccccagaatcacctgggcagctttaaaaactaccgatgccagggccccactattagagattctgatttcattggtccgggatgggggcccggggatcagaattcttaaagagtcgtccagtgattcggaagcactgcagagctgagagcctctgggactggtcccctctcacaattaacctgcaatgatttaggaatctcatgggcctccggccccaccttttgtcgcgggattaagataattatgagagcaacgtgacgtccaagacctcggctctctgcgcatcagaagaagccagggcccggggcgtctaagctcctccctcactccccaaaggaaacccagccgtccccgaagtcacctcgtgggcgcgcagcttgcggatcctgggcgttggccgcgcaggggcctagttttccttggagagacagagggggagtgggggacgcgagggaggcggctgttgccggggcgactggaagcgcgcttccggtgcggaaca

SEQ ID NO: 14382 - RNA, 1023 nt, Homo sapiens
  source 1..1023: mol_type = other RNA
gctgggattacaggcatgagccaccgcgccgggccggaattattgttctttgctctcaattctgtatgacatctaagctccaaaaggaagaaggagaggctgggtaccctgtgccctgagctcagaacttcagggggatgaccggccagtacttgggctgctttcggtcacagtgcttgtcaaagctcagctgcaccgcggcctccatggcttggatcttggcagcactgtccccgtacaaacgcttcatctcggcctggcgccgctcaccaggcctctcagttggggcttctaccgaccggcgggtgttgcagtacaggtcgtggtcagcgttcacatagctgtccaggcgctctgcatccagctgctgctgccgccgtcgttcttctctatgcctctcggtctctgcaaagtactggcggagctcttcagtgatttccatattgctcaggtcacattctacctctgcatctgactcagtctccatctcttcctctttggacaaagcttggtcttcttttgtggatgcctggatcctactgctgtaacgtggatgctgcccagatcttctgaaatgtgaagaactgcaggggtagtcctgccaggccacatgatggtcatagaaggactgaggatacgcagcctcattatcgtaagagctttggggaagaagcgcagaaggtaagtaccatggaagattgaaacaggattccacggccttcctgtaggcattgtgatggctttgcatccaagccattgcttgatgataatgttgccagtatcttgcatataccggatgagaataccaaggcctggtagctttcgatgttgatgcctttaccgctgccatctctgattgtgaaagtccaaatgggtgctgaaactcgtgggcgcgcagcttgcggatcctgggcgttggccgcgcaggggcctagttttccttggagagacagagggggagtgggggacgcgagggaggcggctgttgccggggcgactggaagcgcgcttccggtgcggaac

SEQ ID NO: 14383 - RNA, 1079 nt, Homo sapiens
  source 1..1079: mol_type = other RNA
gctgggattacaggcatgagccaccgcgccgggccggaattattgttctttgctctcaattctgtatgacatctaagctcctgtgccctgagctcagaacttcagggggatgaccggccagtacttgggctgctttcggtcacagtgcttgtcaaagctcagctgcaccgcggcctccatggcttggatcttggcagcactgtccccgtacaaacgcttcatctcggcctggcgccgctcaccaggcctctcagttggggcttctaccgaccggcgggtgttgcagtacaggtcgtggtcagcgttcacatagctgtccaggcgctctgcatccagctgctgctgccgccgtcgttcttctctatgcctctcggtctctgcaaagtactggcggagctcttcagtgatttccatattgctcaggtcacattctacctctgcatctgactcagtctccatctcttcctctttggacaaagcttggtcttcttttgtggatgcctggatcctactgctgtaacgtggatgctgcccagatcttctgaaatgtgaagaactgcaggggtagtcctgccaggccacatgatggtcatagaaggactgaggatacgcagcctcattatcgtaagagctttggggaagaagcgcagaaggtaagtaccatggaagattgaaacaggattccacggccttcctgtaggcattgtgatggctttgcatccaagccattgcttgatgataatgttgccagtatcttgcatataccggatgagaataccaaggcctggtagctttcgatgttgatgcctttaccgctgccatctctgattgtgaaagtccaaatgggtgctgaaactccctgggaatgtctcccactcttttatggcacaagccttcagggactgaacagtaacttttctccaatgggctggtggagctcgtgggcgcgcagcttgcggatcctgggcgttggccgcgcaggggcctagttttccttggagagacagagggggagtgggggacgcgagggaggcggctgttgccggggcgactggaagcgcgcttccggtgcggaacac

SEQ ID NO: 14384 - RNA, 4633 nt, Homo sapiens
  source 1..4633: mol_type = other RNA
gctgggattacaggcatgagccaccgcgccgggccggaattattgttctttgctctcaattctgtatgacatctaagctcctgtgccctgagctcagaacttcagggggatgaccggccagtacttgggctgctttcggtcacagtgcttgtcaaagctcagctgcaccgcggcctccatggcttggatcttggcagcactgtccccgtacaaacgcttcatctcggcctggcgccgctcaccaggcctctcagttggggcttctaccgaccggcgggtgttgcagtacaggtcgtggtcagcgttcacatagctgtccaggcgctctgcatccagctgctgctgccgccgtcgttcttctctatgcctctcggtctctgcaaagtactggcggagctcttcagtgatttccatattgctcaggtcacattctacctctgcatctgactcagtctccatctcttcctctttggacaaagcttggtcttcttttgtggatgcctggatcctactgctgtaacgtggatgctgcccagatcttctgaaatgtgaagaactgcaggggtagtcctgccaggccacatgatggtcatagaaggactgaggatacgcagcctcattatcgtaagagctttggggaagaagcgcagaaggtaagtaccatggaagattgaaacaggattccacggccttcctgtaggcattgtgatggctttgcatccaagccattgcttgatgataatgttgccagtatcttgcatataccggatgagaataccaaggcctggtagctttcgatgttgatgcctttaccgctgccatctctgattgtgaaagtccaaatgggtgctgaaactccctgggaatgtctcccactcttttatggcacaagccttcagggactgaacagtaacttttctccaatgggctggtggagctgaaagaaaagagattggcaatgtcagggaaggccgggatccgcagctctacaaacccggcagccctctccagtgagcacaatggcataatggccaccacccagctgagcccaggcgagtacagagaccattcattgtctgtcctcaaccaccaaagaaggaaggaaaaaaacagggttgaggtcattcactaaacactgacgaggcctataggcaaggcagagactgagtcttgaatgatatatttttccatatagcctctcttaaaaaacggatttacacttcagtacatctgctcatcctgcaggatctatttttaatgcataaatatacacaaagaacaatagataagagctttgtagttttcaatggataaaatgtgactatttccatcaagttaccaaaaaatttcacaaataagtggctttgttgacaggtagtgccatcaaatatattcttttaattacatatttatgttcttataaatatagaatataggacaaatcgtagcaaccaaaaaagtaaaataaaaacacaaattcccctaaaaactagaatgtatacttgaactagattttcctatcttccttttctactagaattctaaaaatacatgaaaattcacctgctttgatctttgcacagaaacacattaaaagccaatcattaaataagttactctggctaaagccctgaaagtcaaaccttccctacaaagctccagtgatttggttctctgaaccaaccaggtaatttggaggatttagttaggtcttcagtacacactgtttcaaggagatctgctggacactgcagcaaaataagtgaaggtatggtgagaaatctgagtgagatagattgagtcatatgcggttccaaggaatctctctgtacatgcaataataaccctatcacagaagatgtcttccaataatacacacaacagtaagaacttcctcactaagacaaagaatataatagggttttgttgagggctgggcttcctgccccacctacttgggcagccctgcccccatccctggctggttgctgaggctggcaagctcatctggcttgatgccctcatggcctccctcctgtgtctttgcatggtccctgcttagtgatttggacatcaaagatggctcaagtccaaatggccttcttccacctgcagacatccaagctccatcttgggcaggacacaggcctactcaagtgcacatgccactgtgttcagaaagcctgcatctccccgtctataatagctacagttaaaactgataggcaagggagccaaaaaactgagttttattttcttttcattccctcaatccccaaccccaatttaccctcttctggatgttgtaataagtactgtcacaaagaaggcatagcatggggaaggagtaaggctgaaaggatgcagttaacaattctttttttcatacaaatgacattccacccacagaagggcattgtttaatttgtcagcaagtgtgatgaatttgtgaatgggtttatttgcaagttctctgaatccccttgtgactaatatcagaatcaaaagtgaaatatgaggccaggaacaaagttaccctctgactcaggaacacaacaagcaatgggatgactgagaatgacataatgataacatagttcaaaagaggaaacagataagtttgtttcacagcaagcatgtccttcataagcaaaacctagtgtgaccataaggtaataagggttgaataggcaggttctgcaaattaagagcataacagcaaaaaccatggctagtttaaagtagttaagatcgctagtacatttcaggcgtcttatttcaaatttacttttttctataaacatattcacggtaattccatgttaatctctcttttctgaatttataggcactcactatgcctcatttacttgggcacttactcagttacctgtaggcatggattctacaatctactccttttaagtttcctattttccttccagcataaaaataatagctaatatttcatgctcttagatgctgctgaaattgttgagcttgtctgttgtttcctgataacgttctctcctcctgcatctactccccaaaatctctgaggacctagtaactcaaaaaactgactataaagcaccaaatcttttcaggaagcaaatatttaaatacattatgttttcaaagatcttttcaattcatctgatatttgatcaactacattcttttttcacttgtccagctgttccgtggctgaatttcctcttgtagagaagttgttcaaaaaaagttctgtacctactttgcaaactctccaatttacactctagccttaactgttcaaaactttcccccgtcattctcatctcaccctatcctttaaaaaaaaacccaaaatgattaatcaccatctatagaacagtttcagaatgaacatttctctctggaactttagtttgtatacttccccagcacagcaatgaacacacagaggggatttatacacctgtgaacttgctttcagttatgcttattccaagttactaaccagcagtctttaaaaatatatggtttctgttcacattgaaattacaaagagactgttattccgataaattatgctagcaaaaatagtatttttaaagggtagctctcatcctacaattcatgggggctgtgagcataaataatcctagaagtgttgcgttactaatctttagtctagattttttaagtaatattgttctgatttgagatgaagaacagctgaatacacagcctagcctgtcaaacgagtttaaaaacatcattcctgaaaaaaataaaattgttcagaaccatctgatctgtactaagggaacatcaagatttcagagctaaaatgcacttcgttggccactggttcaattacagctcattactgataagtgggcagagacacaaggcccataaactgtaggcgccagatgtctcaagataactcccaccaaaagctgacctcctgcagaggttaaagtgcaagagaaaagaaagaaacccgaatttttgagcagagagggcaatatcctagacatccttcaagtatgtggctgtcctgggcgatcttctattcagatactggactggatgggcaaaatccgaattcacctacagaccttaacacggtggttctcggcaccccagaatcacctgggcagctttaaaaactaccgatgccagggccccactattagagattctgatttcattggtccgggatgggggcccggggatcagaattcttaaagagtcgtccagtgattcggaagcactgcagagctgagagcctctgggactggtcccctctcacaattaacctgcaatgatttaggaatctcatgggcctccggccccaccttttgtcgcgggattaagataattatgagagcaacgtgacgtccaagacctcggctctctgcgcatcagaagaagccagggcccggggcgtctaagctcctccctcactccccaaaggaaacccagccgtccccgaagtcacctcgtgggcgcgcagcttgcggatcctgggcgttggccgcgcaggggcctagttttccttggagagacagagggggagtgggggacgcgagggaggcggctgttgccggggcgactggaagcgcgcttccggtgcggaaca

SEQ ID NO: 14385 - RNA, 995 nt, Homo sapiens
  source 1..995: mol_type = other RNA
gctgggattacaggcatgagccaccgcgccgggccggaattattgttctttgctctcaattctgtatgacatctaagctcctgtgccctgagctcagaacttcagggggatgaccggccagtacttgggctgctttcggtcacagtgcttgtcaaagctcagctgcaccgcggcctccatggcttggatcttggcagcactgtccccgtacaaacgcttcatctcggcctggcgccgctcaccaggcctctcagttggggcttctaccgaccggcgggtgttgcagtacaggtcgtggtcagcgttcacatagctgtccaggcgctctgcatccagctgctgctgccgccgtcgttcttctctatgcctctcggtctctgcaaagtactggcggagctcttcagtgatttccatattgctcaggtcacattctacctctgcatctgactcagtctccatctcttcctctttggacaaagcttggtcttcttttgtggatgcctggatcctactgctgtaacgtggatgctgcccagatcttctgaaatgtgaagaactgcaggggtagtcctgccaggccacatgatggtcatagaaggactgaggatacgcagcctcattatcgtaagagctttggggaagaagcgcagaaggtaagtaccatggaagattgaaacaggattccacggccttcctgtaggcattgtgatggctttgcatccaagccattgcttgatgataatgttgccagtatcttgcatataccggatgagaataccaaggcctggtagctttcgatgttgatgcctttaccgctgccatctctgattgtgaaagtccaaatgggtgctgaaactcgtgggcgcgcagcttgcggatcctgggcgttggccgcgcaggggcctagttttccttggagagacagagggggagtgggggacgcgagggaggcggctgttgccggggcgactggaagcgcgcttccggtgcggaac

SEQ ID NO: 14386 - RNA, 2081 nt, Homo sapiens
  source 1..2081: mol_type = other RNA
gctgggattacaggcatgagccaccgcgccgggccggaattattgttctttgctctcaattctgtatgacatctaagctctgtagacataatgagataacaagaataaaaatgtcaggcaggtgattttcattccatgagaggtgcagttggcaaactaccatctgtagaccaaatctggcctgcagtctgtttttgtttttgttttgagacggagtcttgctctttctctaggttggagtgcagtggcgcgatctcagctcactgcaacctctgcctcctgggttcaagcaattcccctgcctcagtctcccacgtagctgggattacaggcacacaccaccatgcccggctcattttttgtattttagtagcgacgggtttcatcatgttggccaggatggtctccatctcctgacctcgtgatctgcccacctcggcctcccaaagtgctgggattacaggcatgaaccattgcgcccggccgcctgtttttataaataaagttttattagaacacagccacacccatttgtttacttactgtctacagctgctttcacactacaaagggagggttgagtagtcacaacactgaccgtgtggcttgcagtgccaaagatattcactctctggccctttatagaacatgcatccctctccactacaggtagtggtatttgtctcactacacacttggctcatttttagtgggggctaatggagctagagtcagagaggatatctggttttttaaaggcatttgtgtagttcagacaggttaaagacaagaaaagataaaaaagcaaaacaccaggcagtatctctaggcaagaacgttaatgaattgaactgttaccaacaacataaaaaaccagtatagtatatgcaaaattattttatgtcaggagaaaatttatcatgttggcaacagaacatgtcctgcagacctccaagtggctggcatagtacatccaccccgtgacaggcccactgggactgtggtgaacatgcctgtaccccagtacaaagtcccctttccctaagaaatgtacagaaggagagataaagagcgtgtacccaaaaggaagaaggagaggctgggtaccctgtgccctgagctcagaacttcagggggatgaccggccagtacttgggctgctttcggtcacagtgcttgtcaaagctcagctgcaccgcggcctccatggcttggatcttggcagcactgtccccgtacaaacgcttcatctcggcctggcgccgctcaccaggcctctcagttggggcttctaccgaccggcgggtgttgcagtacaggtcgtggtcagcgttcacatagctgtccaggcgctctgcatccagctgctgctgccgccgtcgttcttctctatgcctctcggtctctgcaaagtactggcggagctcttcagtgatttccatattgctcaggtcacattctacctctgcatctgactcagtctccatctcttcctctttggacaaagcttggtcttcttttgtggatgcctggatcctactgctgtaacgtggatgctgcccagatcttctgaaatgtgaagaactgcaggggtagtcctgccaggccacatgatggtcatagaaggactgaggatacgcagcctcattatcgtaagagctttggggaagaagcgcagaaggtaagtaccatggaagattgaaacaggattccacggccttcctgtaggcattgtgatggctttgcatccaagccattgcttgatgataatgttgccagtatcttgcatataccggatgagaataccaaggcctggtagctttcgatgttgatgcctttaccgctgccatctctgattgtgaaagtccaaatgggtgctgaaactccctgggaatgtctcccactcttttatggcacaagccttcagggactgaacagtaacttttctccaatgggctggtggagctcgtgggcgcgcagcttgcggatcctgggcgttggccgcgcaggggcctagttttccttggagagacagagggggagtgggggacgcgagggaggcggctgttgccggggcgact

SEQ ID NO: 14387 - RNA, 1999 nt, Homo sapiens
  source 1..1999: mol_type = other RNA
gctgggattacaggcatgagccaccgcgccgggccggaattattgttctttgctctcaattctgtatgacatctaagctctgtagacataatgagataacaagaataaaaatgtcaggcaggtgattttcattccatgagaggtgcagttggcaaactaccatctgtagaccaaatctggcctgcagtctgtttttgtttttgttttgagacggagtcttgctctttctctaggttggagtgcagtggcgcgatctcagctcactgcaacctctgcctcctgggttcaagcaattcccctgcctcagtctcccacgtagctgggattacaggcacacaccaccatgcccggctcattttttgtattttagtagcgacgggtttcatcatgttggccaggatggtctccatctcctgacctcgtgatctgcccacctcggcctcccaaagtgctgggattacaggcatgaaccattgcgcccggccgcctgtttttataaataaagttttattagaacacagccacacccatttgtttacttactgtctacagctgctttcacactacaaagggagggttgagtagtcacaacactgaccgtgtggcttgcagtgccaaagatattcactctctggccctttatagaacatgcatccctctccactacaggtagtggtatttgtctcactacacacttggctcatttttagtgggggctaatggagctagagtcagagaggatatctggttttttaaaggcatttgtgtagttcagacaggttaaagacaagaaaagataaaaaagcaaaacaccaggcagtatctctaggcaagaacgttaatgaattgaactgttaccaacaacataaaaaaccagtatagtatatgcaaaattattttatgtcaggagaaaatttatcatgttggcaacagaacatgtcctgcagacctccaagtggctggcatagtacatccaccccgtgacaggcccactgggactgtggtgaacatgcctgtaccccagtacaaagtcccctttccctaagaaatgtacagaaggagagataaagagcgtgtacccaaaaggaagaaggagaggctgggtaccctgtgccctgagctcagaacttcagggggatgaccggccagtacttgggctgctttcggtcacagtgcttgtcaaagctcagctgcaccgcggcctccatggcttggatcttggcagcactgtccccgtacaaacgcttcatctcggcctggcgccgctcaccaggcctctcagttggggcttctaccgaccggcgggtgttgcagtacaggtcgtggtcagcgttcacatagctgtccaggcgctctgcatccagctgctgctgccgccgtcgttcttctctatgcctctcggtctctgcaaagtactggcggagctcttcagtgatttccatattgctcaggtcacattctacctctgcatctgactcagtctccatctcttcctctttggacaaagcttggtcttcttttgtggatgcctggatcctactgctgtaacgtggatgctgcccagatcttctgaaatgtgaagaactgcaggggtagtcctgccaggccacatgatggtcatagaaggactgaggatacgcagcctcattatcgtaagagctttggggaagaagcgcagaaggtaagtaccatggaagattgaaacaggattccacggccttcctgtaggcattgtgatggctttgcatccaagccattgcttgatgataatgttgccagtatcttgcatataccggatgagaataccaaggcctggtagctttcgatgttgatgcctttaccgctgccatctctgattgtgaaagtccaaatgggtgctgaaactcgtgggcgcgcagcttgcggatcctgggcgttggccgcgcaggggcctagttttccttggagagacagagggggagtgggggacgcgagggaggcggctgttgccggggcgact

SEQ ID NO: 14388 - RNA, 2169 nt, Homo sapiens
  source 1..2169: mol_type = other RNA
gctgggattacaggcatgagccaccgcgccgggccggaattattgttctttgctctcaattctgtatgacatctaagctctgtagacataatgagataacaagaataaaaatgtcaggcaggtgattttcattccatgagaggtgcagttggcaaactaccatctgtagaccaaatctggcctgcagtctgtttttgtttttgttttgagacggagtcttgctctttctctaggttggagtgcagtggcgcgatctcagctcactgcaacctctgcctcctgggttcaagcaattcccctgcctcagtctcccacgtagctgggattacaggcacacaccaccatgcccggctcattttttgtattttagtagcgacgggtttcatcatgttggccaggatggtctccatctcctgacctcgtgatctgcccacctcggcctcccaaagtgctgggattacaggcatgaaccattgcgcccggccgcctgtttttataaataaagttttattagaacacagccacacccatttgtttacttactgtctacagctgctttcacactacaaagggagggttgagtagtcacaacactgaccgtgtggcttgcagtgccaaagatattcactctctggccctttatagaacatgcatccctctccactacaggtagtggtatttgtctcactacacacttggctcatttttagtgggggctaatggagctagagtcagagaggatatctggttttttaaaggcatttgtgtagttcagacaggttaaagacaagaaaagataaaaaagcaaaacaccaggcagtatctctaggcaagaacgttaatgaattgaactgttaccaacaacataaaaaaccagtatagtatatgcaaaattattttatgtcaggagaaaatttatcatgttggcaacagaacatgtcctgcagacctccaagtggctggcatagtacatccaccccgtgacaggcccactgggactgtggtgaacatgcctgtaccccagtacaaagtcccctttccctaagaaatgtacagaaggagagataaagagcgtgtacccaaaaggaagaaggagaggctgggtaccctgtgccctgagctcagaacttcagggggatgaccggccagtacttgggctgctttcggtcacagtgcttgtcaaagctcagctgcaccgcggcctccatggcttggatcttggcagcactgtccccgtacaaacgcttcatctcggcctggcgccgctcaccaggcctctcagttggggcttctaccgaccggcgggtgttgcagtacaggtcgtggtcagcgttcacatagctgtccaggcgctctgcatccagctgctgctgccgccgtcgttcttctctatgcctctcggtctctgcaaagtactggcggagctcttcagtgatttccatattgctcaggtcacattctacctctgcatctgactcagtctccatctcttcctctttggacaaagcttggtcttcttttgtggatgcctggatcctactgctgtaacgtggatgctgcccagatcttctgaaatgtgaagaactgcaggggtagtcctgccaggccacatgatggtcatagaaggactgaggatacgcagcctcattatcgtaagagctttggggaagaagcgcagaaggtaagtaccatggaagattgaaacaggattccacggccttcctgtaggcattgtgatggctttgcatccaagccattgcttgatgataatgttgccagtatcttgcatataccggatgagaataccaaggcctggtagctttcgatgttgatgcctttaccgctgccatctctgattgtgaaagtccaaatgggtgctgaaactctcaaagaaaagagagctgatggttgctgcagatttagatgccctttggtctttaatggtctttaattcgatctttcattcctcacctccctgggaatgtctcccactcttttatggcacaagccttcagggactgaacagtaacttttctccaatgggctggtggagctcgtgggcgcgcagcttgcggatcctgggcgttggccgcgcaggggcctagttttccttggagagacagagggggagtgggggacgcgagggaggcggctgttgccggggcgact

SEQ ID NO: 14389 - RNA, 2491 nt, Homo sapiens
  source 1..2491: mol_type = other RNA
gctgggattacaggcatgagccaccgcgcctagctgagaaaataaattttagaacaattttctggttttgtccatggaaaggctgggaggtagagcagcccagccatcataagcagtcagtgctcagtctgtggcctccaattcccactccctccaattcccactccccactaacgagaaccagggctctggagaaatgggtagttccaggttctgggcaggaaaagtcagaggcagctgtggccccagagcaaggaggcatcaaagcccactggatggaggggctcctctgtccaattacgagataatctgagcatctcctgtttgccaaagatatacgcagcacttgattaaaatgatatcaaatacagttggccctccatttctgtggattcaactgtgtataaaaaatattcctggccgggcatggtggctcacacctgtaatcctagcactttgggaggctgaggtgggtggatcacgaggtcaggagatcgagaccagcctggctaacatggtgaaatcccgtctctactaaaaatacaaaaaattagccaggtgtggtggcgggcgcctgtagtcccagctactcgggaggctgaggcagtagaatggcatgaacccgggaggcagagcttgcagtgagccgagatcgcaccactgcacttcagcctgggcaacagagcgagactccatctcaaaaaataaataaataaataaataaataaaaataaaaatattccccaaaagcccacaataaaaaaccccaaaaatatacagtataacaactgcgtacagagcatttacactgtatcaggtattataagcaatctagagatgacttaaggtatatgtgagaatgtgcataagttgcatgcaaatcccatgccattttatacaagagactcgagcatctgattttggtacccgtgtgggtcctgtaacgcacccctgtggatactgaggacagactgtatacatgaaagcattaagctcgtaacatgagtagggaagcgggaagggtaagtgcagtggtgtgaggaactcccagtcctttggcaccactggagggtgccaggacattcttactccaaaaattgatcattaaagggaaataattaagtgcttatgctgcctttctagtatgaacgcacttcagggtaacctgacttaccctaatggataaagggaaggtctgagagaattccagccactaaatgtccttctgatgagacagaagacgagaattctgcagtcccagtgaaggttctggttctagcaatggtcacccacaggtggcaaaactgtcaggggaacagttgaggggaaactgacgataaaggggtcaggctgtcgccatccaagcttattaatgcttcaacaaagtgacacaattggacatgaggctgtgacacgaggaactgagcaccgtccgggtgtgattccagccacaactttagatccaacttccagacgacaggatatagaggggacagaggaacaagttaaacactacaaggaggatgctaagtccagactggggacaccttcgaggacaagtgaccagcttcaccaacaagtcaagggcacaggggagggaagagggggacttttaggatcaaaaggatcctaaaagactttgtagccaaacacaaacgtgaataaagctttgataatccaatcgtgtgaggatatttcttaggcagtaagggaaatacgaataggactgttagagaacattacagaattcttatgcattttgtgaaaacagcactgtgccgtcagttattgacttcttgtctcttggcttgtctgtgctctgccctgagtgctgcccttccacacacccttccagctgggtgtgctggagccctggatgcaggagttggggctgggacctccctggtgttcccaggttatttcagcatcactttgggagcagagacagctctgagcccagccaccaggtcccttggtgcccccttggctcctggagtacagtcctaggccctcctgcccctcttgcgagaaccaagcacatcctgtaagctctgaggtccctgaaaccccaccctggtaatactttttgtccccaagccctggaggtggtacctgcggttgctaccctggatgttaaccctgcgcagcctgtgtgctacctattctgactctgcttcccaacacccgtgtagcctcgtctccatgtgcctggtgagacttctgatatggcaacgagttaagagaaagaaaatggctttgtgttgttttgtgatgcctaccaaaggatttaggggcaagtgacaatatgtctggaatttgcttacgtgtattcccgcagaagtgggggaggaaaagatggaagtgctttgggcaaaatgctggcaggtgctgaagctgggtgacaggtacaagggtttagtgtatgtttggaaactttcatagtgaaaaaaaccccacaaaaacgaaagctgtattagagttacaaactaaa

SEQ ID NO: 14390 - RNA, 241 nt, Homo sapiens
  source 1..241: mol_type = other RNA
gctgggattacaggcatgagccaccgcgcctgaccccgatgagccattttggacccagggctttgtctgtcaggtgtgttggatgaagcccagttatatgcttaagtctctggcttcatcctgtcatcccaatttggaagcccattaagaaagtgagctctgttttgtttttagtgatcactacattttcccctaaactcagagaaagatctatgagcacgtaaagcatcaaggttgtggc

SEQ ID NO: 14391 - RNA, 3848 nt, Homo sapiens
  source 1..3848: mol_type = other RNA
gctgggattacaggcatgagccaccgcgcctggcacacacacaagaccttttaagggtgaacaacctttatcccacgtatatggcaatatagatataataagcaaatgatataacaagcaaattgcagtggaaaggagtgaagggaaaagatatgtccatatatatttacaccaccagattatggaggaagcatcaccagactgggaagcaacagcctgggctccagagtgggccgccggtccgtgcacagacgaggagaggtctcatggagcttcagtgcggtctgggaccctagctcttttgtaatgaattgtttggcatgaggcccagtcacgagggcccttcgagactgggctcaagggacacaaaaaggtctacttgtttttgtgattgtctgttgtttctcagtaactgacgtacaggagcagatttctctaaaactttgctggatgaatgcctcaaggggctcatgcaacctgttccgggagttggtgaccattgtttatgtccatgttcaattgagttcaaattaaatatttaacttttcctccacattcggcctcaatttgatactcagttgtggataaaacgtgtaaagatacatggggaaggcatagttgatatagattacagatacagggtaaacacaggagaattaaaagcacaattaataaaaaccacacccaccacggccaacgccaatgccagtcggacagccaattcacgatggggtgcccatggttatattctaactgctttgtttttgcatgtcttgggcaaggagagtaatattgtgagaattgtcagggatatacacacaacattcagcatgcagtaaggcgcaaacccttccttgggctgctgtaaggatgtgtaatgccatttgattttgcaacacaacagtacgcccctgagcaaattcatctgataacaatgtaagtccagtgctactagcattaagagctttttctacatgcaagcttagtattttaatttgttgttgaagcaggattgtaccagcagtgatatggtaccaccaccagggagtccggcgcatttgtaaccagcaatatttgtaagtaactagattactggggagggaaatattatcccagatagtgaatggaattaatggccacccccaagtgcatctccctgttcagttcgggggcaagtatcaccacccataggatccgcatacccagagggccccccagggaaggggaagagttctactacaatcgtattgctgtaatgtgtaatttaagtaacaaaggtgctgtgtttcactgggggcactgttattgatttggaatatgtgctgacaactgtctggtgggagaaaccccagagtgtcattggggaagccatttaaggcccccaaacaaagggggggccataaggagtccagctaccagtatgacaggttccccgtatacgctgttccaggcatatcaggtaggatacaaaagcttttgactcattgcaagggtggatttcgccttttgttgaatttgggcaagaatagactgtttagtttggttaaaagaagttcaggttgtactacaggtgctattctcccaaccccattggtagcgacatagccacttggaaatattagcagagataatattctaaggtaatccattccctgcagcctctggcaactcgacacataccagcactgactgcggttgagctcttttgcagcagtggctaccaggtaataaattcattctaggcctcagacacaaagacacaagacacatcagtagataggtcattccctgtaatagcaaaagtggaggggaacatgatattgttttttcatatttaggaaattgtactatgccttcattttctgctcccatagctacaaggtcaccagcctgaggggtgggatctgatggacgctgtacctatattttggctccaggatttaagccactagtaccagtggatctgaataacctggttctgtatgtagcctctgttggggcagagatttcctacagggttaattgctgacaaggtaccactaacaattgagcaactggtatctgcagttttatagcaaaagaatctggagtggtattgtataaaatgacctttaactctccccggtaatcactgtcagttatacccccgtgtactgtaataccccgcattgcaagacctgattggaatgtaatccacccataatgtttgcaaggtataatacctataataactcctaagccggtggctaccgtgtatgtactttgggcgggaattatcccaggctttaaactatataagtccaaactggcagctcctcttgtactcctccatgggagtgggtggattttccagcatttcagcaagagagggtggactacacctgcacacttagcaatttgtaagtgtaggataagcatttggctcagtggggtttcagatgttgttaatggccgattatttaaaatttgtactatctcaaacaggtgatcgttccatttttttaacttaccttgccctaacacctttagctgttttttcaataacccgttcattctttcgattaggccagctgcctgtgggtggcatgggatgtggaaaatccattctatgccatgttgggctgcaaaggtttgtacagccttacctttgaaatgggagccactgtccatttgaatttgtatgggcacaccataatatagaattaggatgtttaaggttttaatagtgttagtttggttagcattagcataagcgcaggctactaggaaccctgagcaggtgtctacagaagtacatatgtattggcaccctttagaagtggcaaaggacaagtatagtccatttgccaaatttgtcctggcatttttcccctatgaatgtgccccaaaaccctctgaggaactggcttagtttttaactgttggcgtgtagtgcgttgggataaagttgtgtgaaccacatccttcggtaatgatatccctctttgctgtccccaagccatggttccctggatgcctagatgtcctcactggagatgcacccattgcatgagcgcagcccaatccggttcttctgggcctgagtctgcagtaatagtggaaattttagcttgttggtcagccttctgattagtctgagattggtcccgggtttgtctgccccactccttaatcctctcctccccacagggcatccgatcccccaagtcctgtagctgacctagttgttccagtacctcccgtgtgggagtatcagactatggaggaaggatcactagaccgggaagcaacaatctgggttccagagtcggctgccagtctgtgcacagacgaggaaaggtctcatggagcttcagcacggcctgggaacctagctcttttgtaacgagttgtttggcatgaggcccagtcatgagggcccttcatgactgggctcaaggaacacaaaaaggtcaacttgtttttgcagctgtccgttgtttttcaataactaacgtacaggagcagatttctccgaaactttgctggatgaatgcctcaaggggctcatgcaatctgttctggggcttagtgaccattgtttatgtccacgttcaatggagttcaaatttaatatttaacttttcctctgcagcaggcagccgcaagggaaggtcacaggtaggctggaagcccatggcaagagctgaagcttgatgatgtccttcagctgcagtcaggaagaaagttctaaggggaaaggagagcaattgttgacccagcagctacttggaggatctccctcagagaaggcccatttttaaggagctcaagtcaggcccacccatgataatctcccattaattaac

SEQ ID NO: 14392 - RNA, 4415 nt, Homo sapiens
  source 1..4415: mol_type = other RNA
gctgggattacaggcatgagccaccgcgcctggccaatactaaattttaattagaagttagtgagaatgaagacctaattttccatccgacttcatagattgaattctgtctatggaacccagtttgagaacccctagtttaacaagtgatttacacctagtgtgaaatttttaatcagatttatttcagttaactctgagactaccccctcacacacaggaaggtgaaaagaaggcttggagcaccagctagggaggacagggaggacaggaaggcctctgagggtgggcagagctggagaatggacgcaaaatcaagatgggaaggagccgcctcaagatttcatgggtgtggtggtgggggacctggtttagcttctctcctgttctagacagctctacagagacagagctcaagggagcgttttctacaggttccccgtccggaatgcccagctcctatgggccctaactgaggcactagaggaaggatggacgagcagagccaggagtgggcacgcctttgtgcccagccttctaggtctcctgggttgggcaggacacagagcaaaaccccttccccaactcacacagctccagtcagctgctggctgttggcagggcaaggcccaccccccagagcccaccccccacaagctgtcctctgagacctcactgccacaagggtgaactcccacccagggttctgggctttgcttcagggtgctttgctctctgcccagaaaaacatcccccagaaaaggaaagacaaaggggtggttacctgctgacctccccacaggtttaccctgaaccgaggcccagagaggggaagggacctggccgaggtctccaggaggtcggggatgtgctggtgccctgccagccctgggcttctgccctctcctcccctcagaccagctcccaggggaatgtgaagaaaggagggccacaggcaccagtgaggccaccctggggacaaacaggtggttagaggcagctcagacctcagacattatccagggcacttttataaacaggaaaaatgtggccgggcaaagagtagaggctcctgctaacaccaccagctggtaggtggtgaaaccgcacattagcccttggatacgtgattccccagcctgaccatgtattagaatcacctggattgctcactcaaaacatgtctgctggcatcaggcctgacgctacagaatcagcagctctgtagaggggcctagcatctgcaccatcaatgagcagcccagatagctccagtgtgcagccaggtttggggcccatggcactgagccattcccaagtatagcctaggaagagatcctgagctgtgggcagagggagggaagagctcggggagagcatctggttcaagacacttgattcacttctttttgttggttacatctaaaactaaggatgggtggctggggcgggagccagaatttagtcttagctgagctgggggccaagtggagtgtgccctgaggcttgggacaggagcatgtgggtgggacttcccatccctgacccccacccttatcctgcccttcagtggctatgagagatggcaaccaggtcacagggctggactttgtcgtctcaagccccaaggagtaaagctgggcagggctttggcctggatcaatggccttaggactcagcccacacgtaagtggggtgagtgcagcgcaggacagcgtctgtgttctccagaatctgtcttcactctgactcaatcaccaggggattctgcaccccggtcttagtagaaatgcacctctgagtttcagtttagctccctgcccatcacgtcaccacagtggtccatggaatctgatgcgtcccgcagctcagcccttccaccttgcccagtgtgccctcctcaccgacagctcccgctcccagccccctgcctctccacttctagggctgcaatctgcttctgtctcctccttggatcacacacttggacccagctccctgttttgctctgggctctgctttctcttgtggagttggtgtcaccaaggtctcaggtgagaaactccttcctgccgtgtgactgtctgcggagaagtggggcaccctgtgggggatgggataaaaggggtgtccatgcactccaagctgtggccccttgggttatagatcagtttttatccaaagacccttgtgatgagtccaggcttgagtttagtccctattccaagacatgagtttgcatttcttctttcattggaagatgacatttcaaaaactttccttggctttcaaaaagcttagcattagatgatagaaatcagctcatgggccccttgcttttaggtgatgtttattctgtttcatccttgaatatcaatttgtcgtgcatccaaactcgctatgtcaaaccttttgaatgaatgcagggtatacgtcttaaattaactccataaaacttgagtagctagcatagaaatttaaggagtatgtgagcaggacgttatttcccccagttcacctggccttcttgcactcagtgctttcagcagctgtagggcgttttgtgtgaagttattgacatgaagggatgggagtgaaatcagttatcagataacaaacaagtgctctcatgtctgatgggtagaagagggggcagtcacttcctcaacacgtgagatgacactgactttgcagtgagctctccccaggaaagaggaggagccctgggcaggcgggatggggaaggaccctgcgggaaccatggaggaagtttggagctccctgctggagcatgcagcctgcagggctgcagacagaaaacctcgttccgccctggtttggaggtttgctggctgtgtgaaccttgacaatgtacctctcctctctgaatgtcagttttctcaactgtataaaggaaacagtaatagctactttggttgtttgtgagggtcaaacgcaacacacatacagaagccctataaaatgcaaatacttttatcctcagttctgtgcagaggccactgggtttacttatgtattgattctctctgtcctctctcccacccctatcctcctccccacatgccctcaccttcttggttttgccctcccagaagtaggggagtacagttattcggttagagcagttacactcttgggggtttgcttcagccaagaagacagtgagccgtggggatcgtaattaatggaggcagactgattagaaatgagccactggatcggggtgtttgctgattcatcttggaaacactaggtcctgagtcccaatcggcttctaccacattggtcattgttctacttctgcactgttctgtgcagaagcacctgtgtttactcataaacttacatattgattctgtctcttctcctacccccatcctcctcctcatatcctaagtgctcagcatggtgctaggtacacagcaggcactaaataaatgtttctttaattaaattcccattgatagctacactgtgtgaatggtactttcatgatagatttttctgtcaccccttgagtttctgcagacattaggattcacagagaatgctgtgttccaagtcaaaatattcattatgacacatgctgtttgcaatttccacaatccaagtcattacccataatgtgcttggggaggaaaacaaacctctcttggaaatgctgccgtgtaggggttggggtcagagctctgcctccaaactccgtgacctttcctggagcacttctctgttgaccgtgaccaggaggcattccaggcttgggagcaccagccagaggacccccagccagatgagatccagtcacacatctcaggcaaggtcagacagcccagggaccccaggaatgcagcccaccagatgtgtgctaaggacagcatgcttatttggaacgctgggtaacctgtcatgcattgcagaaacatggagatccccctgtttgacattttctcctgttaatcccattttttaaaaatagctgtgcggtgtagaagtttcctcctggtctcattaggtgtctccttataattgcaggttttaaagcaagctcaaggcagagcctttcagagaaattaaacttcaggtgttgtctaggaccaggggcagccaattatcccattacagaaaccatgtacttggaatactgattgtgcttcagaataatccaattccattcactgtgggctgggggatgcgcctggcaatagaatttcaatagcgaagagtctcagtttatcctcatgaagctttcagtcttcttcctggggttagttcccttcttcttgaaatatattcactagaagttcctcagtggggatattttggtggtaacagggtcaggactagagtgaggcacagttccatatggctggggaggcctcacaatcatggtggaa

SEQ ID NO: 14393 - RNA, 1645 nt, Homo sapiens
  source 1..1645: mol_type = other RNA
gctgggattacaggcatgagccaccgcgcctggccagaagtaacttcttaggatcagagatctttaggtactttgcatcccaaatttctttattttgtgaccagaagaaaatattaaaaagaaaaaaaaattttttaaacagttccattagagcaaagcatcaaaaaatcctgttccatttgaggtaggatgttagctgctcacactgaccctgatccccaaggcttcgtagaatcctcctgctctgaagtagtgtcaggcataattatttttttgcttttcttttttaaactacaagctttatgtgcatggtttggtcctcatgttgctgccctagctccggggcagatcattatccgaggacaccatcttgcattgcactaagaggtcattattaatgtctcagcaattaagctccttcccccaggctggtccactgaggtgacactgcggcaaccctgaaatcacatgttccattgcagagagcactacacaatactctctggtacttggatgtgcttttcttctaattttgaatgttgtacattttccttcctctttgtttttgcttctgagtacaactttgtgatgtagttcatgcaacgcatagggtgggaagattggccatttttctcttcagatgatgtttcttcattatttgaccttgatctgtaactttctagtgtgtgttctgaaacttcgttttctttcttccatatcacatgtgctttcctcagcttcatgatgaagagctggactatgatgaagagtatgaaaatgaggaaggacaccagcgtgagcagcaggatgccacttttctttcttgccagtcctaaatactgaggatttgcttcggtggtcaagtcaggatcttgagtggtttgttctttctcttccttgtcaatctccgatgtactagaatcttccgttactgagacagtactggtgggctgctgtgggtcttgagaggatagagagtttctctccagagcatctgaagctgtctcttcatcagtaaccaaatcttcaaaccggaagggtgctactagttttctcccttgcaggcctctgtgtcggataatgcagtccaccgttgaatttttgccataagtgtggattatgagagtgctggtagtattacatttcttcccatcagtttcaaattcatggagcgttccaccggacacttccatgctattcccaagtagccaggttatctgcggagggggcttgcttctcatggtggagcacatgagtacaacatgttcttctccattttgctttctgataactgaagcttccaggattggcttgaaaggagttgcaggatactcatttaaaaaaatggtgaaccctgagggggtcagccactggagggaggagttcttcctcagagaagtgacacactttagagtgagcgtctggccttcctccacggtgatggtttctgtgtggttagtcagagaggcctcttgcaaggggaaccatgccagcaagctgagaactctccaccacatactgtgctgtgctgctgtggcacctttgtcaacttcctctagattctgagacaaatggagctgagtagtttcttttaaagggggagaggcagtagatctgtgacctcatgtgtatcaactcctccatc

SEQ ID NO: 14394 - RNA, 1717 nt, Homo sapiens
  source 1..1717: mol_type = other RNA
gctgggattacaggcatgagccaccgcgcctggccagaagtaacttcttaggatcagagatctttaggtactttgcatcccaaatttctttattttgtgaccagaagaaaatattaaaaagaaaaaaaaattttttaaacagttccattagagcaaagcatcaaaaaatcctgttccatttgaggtaggatgttagctgctcacactgaccctgatccccaaggcttcgtagaatcctcctgctctgaagtagtgtcaggcataattatttttttgcttttcttttttaaactacaagctttatgtgcatggtttggtcctcatgttgctgccctagctccggggcagatcattatccgaggacaccatcttgcattgcactaagaggtcattattaatgtctcagcaattaagctccttcccccaggctggtccactgaggtgacactgcggcaaccctgaaatcacatgttccattgcagagagcactacacaatactctctggtacttggatgtgcttttcttctaattttgaatgttgtacattttccttcctctttgtttttgcttctgagtacaactttgtgatgtagttcatgcaacgcatagggtgggaagattggccatttttctcttcagatgatgtttcttcattatttgaccttgatctgtaactttctagtgtgtgttctgaaacttcgttttctttcttccatatcacatgtgctttcctcagcttcatgatgaagagctggactatgatgaagagtatgaaaatgaggaaggacaccagcgtgagcagcaggatgccacttttctttcttgccagtcctaaatactgaggatttgcttcggtggtcaagtcaggatcttgagtggtttgttctttctcttccttgtcaatctccgatgtactagaatcttccgttactgagacagtactggtgggctgctgtgggtcttgagaggatagagagtttctctccagagcatctgaagctgtctcttcatcagtaaccaaatcttcaaaccggaagggtgctactagttttctcccttgcaggcctctgtgtcggataatgcagtccaccgttgaatttttgccataagtgtggattatgagagtgctggtagtattacatttcttcccatcagtttcaaattcatggagcgttccaccggacacttccatgctattcccaagtagccaggttatctgcggagggggcttgcttctcatggtggagcacatgagtacaacatgttcttctccattttgctttctgataactgaagcttccaggattggcttgaaaggagttgccagcacaatcactttcacttcctttgtgcttacagagtcgctgtaatgtaagcacttgtacacgccttcatcttgcagggttacgttaggcacagtgatggagagctgattggccgagtgatgaagaagctggtatttggaattttttaaagcaggatactcatttaaaaaaatggtgaaccctgagggggtcagccactggagggaggagttcttcctcagagaagtgacacactttagagtgagcgtctggccttcctccacggtgatggtttctgtgtggttagtcagagaggcctcttgcaaggggaaccatgccagcaagctgagaactctccaccacatactgtgctgtgctgctgtggcacctttgtcaacttcctctagattct

SEQ ID NO: 14395 - RNA, 1151 nt, Homo sapiens
  source 1..1151: mol_type = other RNA
gctgggattacaggcatgagccaccgcgcctggccagaagtaacttcttaggatcagagatctttaggtactttgcatcccaaatttctttattttgtgaccagaagaaaatattaaaaagaaaaaaaaattttttaaacagttccattagagcaaagcatcaaaaaatcctgttccatttgaggtaggatgttagctgctcacactgaccctgatccccaaggcttcgtagaatcctcctgctctgaagtagtgtcaggcataattatttttttgcttttcttttttaaactacaagctttatgtgcatggtttggtcctcatgttgctgccctagctccggggcagatcattatccgaggacaccatcttgcattgcactaagaggtcattattaatgtctcagcaattaagctccttcccccaggctggtccactgaggtgacactgcggcaaccctgaaatcacatgttccattgcagagagcactacacaatactctctggtacttggatgtgcttttcttctaattttgaatgttgtacattttccttcctctttgtttttgcttctgagtacaactttgtgatgtagttcatgcaacgcatagggtgggaagattggccatttttctcttcagatgatgtttcttcattatttgaccttgatctgtaactttctagtgtgtgttctgaaacttcgttttctttcttccatatcacatgtgctttcctcagcttcatgatgaagagctggactatgatgaagagtatgaaaatgaggaaggacaccagcgtgagcagcaggatgccacttttctttcttgccagtcctaaatactgaggatttgcttcggtggtcaagtcaggatcttgagtggtttgttctttctcttccttgtcaatctccgatgtactagaatcttccgttactgagacagtactggtgggctgctgtgggtcttgagaggatagagagtttctctccagagcatctgaagctgtctcttcatcagtaactaggaaaggggaaaaacaaaattctgctactatagagagcagttttacccacattgtgctcagtaaaagagattggagaatatatttagcggctacctgcttgtagaggttgtgcagaaaccccagaactgt

SEQ ID NO: 14396 - RNA, 969 nt, Homo sapiens
  source 1..969: mol_type = other RNA
gctgggattacaggcatgagccaccgcgcctggccagcatgggctcttgaaccttcctaaagggatatctaatactcaccaacagtggggcaagtagtcccacttccaaaaccttcctagattgcctgacatgaaggccactgattggttcattacaaatttgctgcaaaaacgtaaggcctgcataggccactgccatgagaaggcagcccataggtgacggaaagccaatggtcctgcctgtcacatttgcctgagatgaatggctttcatttccccaagccaccgagacatcatcacccacagcacctctgcccgagtttaatttcacatcatgcagctttcacaaatgagtgactgtgggcagtgtttatcgaggaaatctttttgtagccaccaaacctgtggaaccactttcttctttaatttccgtcccgtacttccttgggaacagcagagaaacaggtggcgagctggatctggccatggccataatttatagactttgttgtagagtagagtggtggccagagaagaggagttcacggtgctcgtcaccagcttggactctggaattccaactcctcagtttatcacttctgtgacccctgagagttgccttgcttctttgagcttcagccttcccctctgtaaagtgggaataataacagcacctctcattgcgcatttaattttctccaaatataaatcctccaacacatatcctggcacatggatctttgtgcgtatatcccagtatttcgtaggttattgcctgtaaggaaaattgtttgagtccaaggttatgctcactcaaaggtgttgctacagaatcctggcacccctcaccagtgtaggagagggcttgtctctccaccctctagcccacagagctgtcatctttcttaaccttggccaatctaaaaattataataaaatggccagggaaaattatagtaaaatgacatc

SEQ ID NO: 14397 - RNA, 1308 nt, Homo sapiens
  source 1..1308: mol_type = other RNA
gctgggattacaggcatgagccaccgcgcctggccagcatgggctcttgaaccttcctaaagggatatctaatactcaccaacagtggggcaagtagtcccacttccaaaaccttcctagattgcctgacatgaaggccactgattggttcattacaaatttgctgcaaaaacgtaaggcctgcataggccactgccatgagaaggcagcccataggtgacggaaagccaatggtcctgcctgtcacatttgcctgagatgaatggctttcatttccccaagccaccgagacatcatcacccacagcacctctgcccgagtttaatttcacatcatgcagctttcacaaatgagtgactgtgggcagtgtttatcgaggaaatctttttgtagccaccaaacctgtggaaccactttcttctttaatttccgtcccgtacttccttgtggaaaagagccgggtcaagagaaggggcgtgtttctcccagtgtattcggcaagtaatggagtgagcactagtgagggtgagacctgtccctgcaacgattccttcccatctcctccaagtgctctcccccaccatagcctctgcaggtcctggctttgacattcactcgccgtgtgactttaatggggtcctttgcctttctgtgtgtcagttttcccatcttgggaacagcagagaaacaggtggcgagctggatctggccatggccataatttatagactttgttgtagagtagagtggtggccagagaagaggagttcacggtgctcgtcaccagcttggactctggaattccaactcctcagtttatcacttctgtgacccctgagagttgccttgcttctttgagcttcagccttcccctctgtaaagtgggaataataacagcacctctcattgcgcatttaattttctccaaatataaatcctccaacacatatcctggcacatggatctttgtgcgtatatcccagtatttcgtaggttattgccagtgaggctaaatttattccaatatcagacagtttcagtccatcttaggcatattacatcaattactatggtgtccctaagagcacaaaataccccagggggggttcaaaccagcatagatttcagaggcatctgctcaacgggtctcagctaagtggttaacggtccccacagggtgctgcccagccaccagggcctaaaatgtgctcagactccagacatggaacaagactgtctggttaatagcacatgtggcccagccaccccagtgtggcatttacagctctctggtttctgtcaatgctg

SEQ ID NO: 14398 - RNA, 5083 nt, Homo sapiens
  source 1..5083: mol_type = other RNA
gctgggattacaggcatgagccaccgcgcctggccaggactaactcttaaacatgaataagaactaaaagtaagctagatctgattctataataaccttacaaaacaacaaatttacaaaaatgaattcacaaattgagctcatacctacttaaatatatcgttatacttctcagtatttacaatatgtatattcacaaagtaaatgttgttacagacacagaaaaacatcaagcccccctgctgtgtttaaaaataaataaaacctaaatttaaaccgtgtgtctcatgatctatgtgctctgcagtctaatgttccgcatgtctctcagcagcactgttcggtagttttgttccaaaatttccatgtattcaaaataatcactcactcgaaacccatgcagtgcttcttcttttaggaaaacttgcagatcttgagtctgagtgtgctgtagaatgtcttgctgtaaatgtttgaatacagctatacagatatacacttgataatcaggaccaaggaaaacacaagtagcaatataatggcagatttctatccaatctaagtaattccaaaaacactgggttatccattgcaggcaaatctgtgatggtgcaaaaccagacatgtgaaaagctgaaaacacaagaggcaactcagccttcagtagcatttcaatataatgggtgctgcaaaaatatactggatggatgccagattctacagtgtcattaggaaggtaactagaaatatgtagccttggcaaccaaagaaaagcagaagtcagaagcctggagaattgatgaagaaattggaatgttttttctttgtctcccaacattatcatgaacagagaagatacaaaccagtcatggccagcataattcccttgcaggcagagaagagaagattttatggaagtttgctgctgtttcaggaatctctcacaatgctttaaaacccaggtaagatcattttctgcaccatcttttaagagactgaggaatttgccatacctgacagtcattttaatgccaagctgctgcacagatgaaagactttcattcttcacatttgcatcagtagctaaagacaacagaaaactgagttataaagtgcagaaaagtttgcataataatcacattttaattgaaaattgatgaaagcaatatttttacatattttaatgtgaattttgaaaacactgatgaatttattcttttaggaactgtcagttacattttcaaaggaattaacagaaaactttttacaaataactttttcccataaaaagcattggaaaacatattaaatacataacaatagtagttttaaaacaatctattttacttggctctcagaataaaaagagccattgacccaaaaagtggtctagaaatactactttcatcatgcaatgcatacataaaactctgaattacaaatatatacaagaatggttatttcgttcctgatactaatctttaagtaatcagtgttccacttttaatgtatggtaacgtatgagggtagaatgaatgaatttcttcctgcaggccaagttttctttgcgaagtagttgttgtaatcatctgtatactccactgaagggaagtagcattcagatgggctttcagtgagatgaagcacaaatttttcaagtaattctattaaggcctctccactgattatatcaggtttggctttcatcattttgcaaaattgtctttggcagttttctatccattcagtttgtttatcagatattttgaggcataataaaagcttgtcaagatcattgttcactgaacgctgcatagctccagagacacagaatatggtattcttgttctttggccccatctcttgttttataccagcatttcttgtaatgtctgacagatagcagtttggcaatggatatgatgaaaacattggccaaggatatggattatcactcttttcgagtaacctcggaggcaaaatccgttccaatggcccaccaacaagatttattctaacaagaacatgatttctctccactgataagccatcaattataaagtccctgtggctctcagaaatctccaagatattttcttcttgagcatttagtaacatttcagatacctgatactgagcctctaacaggagaagagtgtccagatcacagcatatcacacttaataacctttgaccatatgtggagaaccaaggaacataatgaagttggttggttgctcctaagttcagtggacaaagtaatgaaagaaaatgatgaactctgggattctgtctcctggcttcagaagctgaggctcaaatccgctaagattgcccatagtgagtggcttatttccttagaccaaagatatgtgattgttcatagttgaataaagaacgaatcttagcttcagaattcaaaattataagtctatcaataatatcaataacacatgttgggacttcacgaagagaatattctgttttattaggaagatcttgattccttacaagctcataaatagcaggataggataacaagttcaccagtgctaaaaaagattgcaactgtaaagtttactgctttacattttctaaaaattttcactagagtcagaaacttggagaaccagacatactgagatatttcacttttgacagcttcggtcaataggatccactggagtagttctgggatgggttaccctaacatcatctcttccatattccagattggaccataattcagttataagttcattaataaaccctgacttttttagtgcaatgccacctgctgctgttgatgccactcgtgtaaccaaaactccatagccaaattttttatgcctgctgacctgtaatttttttgcatatcgattgaatataaatgtcacacattcattgatagcacctgttctttgaagaagtagtaatcctttgggggtggcagcaaaatgtagtaaatcatctaacaaattatcttcccaagccataatgttttgggattcctggcttactgaagaaacagaatcagaaccctctactggagtaggaattctttctgatagcaaacttgtctttttccatgcctttgctatagattcatgcaaattataagtgattaacacctgcaaaccttcacatgtactatatatgtgacgacacacagaaataaaagctcctttaaccacaggcaacatttctgatccagaaaatatagaaatatcttcatcgagaagttttttcgaaaactgggcaattatatgagcacctgtaggactttcttcagaagagttcatatttgctccataaaggagtaaaataagcccttcttctacagatgcaattcttgccaaaataccagctatatgaattaaagctgtctcagagcaatttggagatgcctcatttcctttcattaaattgtgaataggctgaagaagtgtctctattacaatgttgttatataagcattccactgcacattctttttgatcactgagtatccacagaacttcagtcaccatacttgcaggagagtaattctctgaatgggcagctgatgtcatctttggacaacttggtgagtaatagataagttgggtaaaaagaacaagcagatctatgagggataccaaaccttttttattcttcagcttaataggaaatagttttctgccttgtttatagatcaataatcttcctaaaaggcacagtgagtgaatgaaataaatatattgtaattcttgtcctaagtagtagaaagttttctgcttgtttctgcaatgctttgaatgtcccaaagtttcatcagctttcctagtcttacacatttcaaagtactgaacacactgttgaatggctgtagttaccagagacttatatttcgtttcaagaagtcttaatactgtagttctgctataatgtgcatgcatccactttttgaaccacacagccttggtatcaactaatgcaaaaaagtagatcggatccaaaatcttttgtgagacaacatggctttgattatgtttaactgttaacaaggacaaagtactctccacaatttcttccatatacttctctggatgacgaatccagaaagatggagcttctttctgatattcatttagaagacgaacctttttaagtaagcgagtcatattaggattagttatatctacaccagctgaaagagtaggaatatgattttccctagaaagaaagtatgactccaaatacttagctaagcttgtataaatttccttggtcatatgtaatggagaaagcaaaaatgtctgtgcacagaattttaaaatccggtcactaaacacaggatcaggatctgaaagagacacggtcagtttttcgcagagagtagtccaattttcacagttgaggacatcagatggaggagctgaacataatgtttgcaaggcttcatatctcacctctttaggttgcccaggatccaactggtctaaaatcaattgtaattttccttgacaaaatttgtaactctgattcaatgatgaatcactatcagagcaattgtctgtgcggtaactatggcttttctccttttggatttttttctgcctttcttgatttcgtgtctcatcttcttcaaacttgttaatcatagactcgaccacagctatcataatgttcttcaggtaatgcatcatttctttgtacctttaaattcaaggtagttctttagattcttgagttcttttagtgacctgctgtacaactgtatcatagccgcattcttcaccctgattccgatcagatgtgcatttttccatttcttcttcaatcatagaacccaaagtgttgcctatatgctgcctgaggtatttcacaaattcatagttgtgaaaattttcatcagtttcctccagatgtaaaagaatctcttcggcacactccagggaaggggcacccgtgattttctccttcacgctctggaacaaccgcctcagcatcgcctgcagcatcgcctggtcctcgctggagaaatgggccatcctgttggaatcaaacgtccactctcattactccaggtccgagcaaaagc

SEQ ID NO: 14399 - RNA, 4239 nt, Homo sapiens
  source 1..4239: mol_type = other RNA
gctgggattacaggcatgagccaccgcgcctggccaggactaactcttaaacatgaataagaactaaaagtaagctagatctgattctataataaccttacaaaacaacaaatttacaaaaatgaattcacaaattgagctcatacctacttaaatatatcgttatacttctcagtatttacaatatgtatattcacaaagtaaatgttgttacagacacagaaaaacatcaagcccccctgctgtgtttaaaaataaataaaacctaaatttaaaccgtgtgtctcatgatctatgtgctctgcagtctaatgttccgcatgtctctcagcagcactgttcggtagttttgttccaaaatttccatgtattcaaaataatcactcactcgaaacccatgcagtgcttcttcttttaggaaaacttgcagatcttgagtctgagtgtgctgtagaatgtcttgctgtaaatgtttgaatacagctatacagatatacacttgataatcaggaccaaggaaaacacaagtagcaatataatggcagatttctatccaatctaagtaattccaaaaacactgggttatccattgcaggcaaatctgtgatggtgcaaaaccagacatgtgaaaagctgaaaacacaagaggcaactcagccttcagtagcatttcaatataatgggtgctgcaaaaatatactggatggatgccagattctacagtgtcattaggaaggtaactagaaatatgtagccttggcaaccaaagaaaagcagaagtcagaagcctggagaattgatgaagaaattggaatgttttttctttgtctcccaacattatcatgaacagagaagatacaaaccagtcatggccagcataattcccttgcaggcagagaagagaagattttatggaagtttgctgctgtttcaggaatctctcacaatgctttaaaacccaggtaagatcattttctgcaccatcttttaagagactgaggaatttgccatacctgacagtcattttaatgccaagctgctgcacagatgaaagactttcattcttcacatttgcatcagtagctgtatactccactgaagggaagtagcattcagatgggctttcagtgagatgaagcacaaatttttcaagtaattctattaaggcctctccactgattatatcaggtttggctttcatcattttgcaaaattgtctttggcagttttctatccattcagtttgtttatcagatattttgaggcataataaaagcttgtcaagatcattgtcttgttttataccagcatttcttgtaatgtctgacagatagcagtttggcaatggatatgatgaaaacattggccaaggatatggattatcactcttttcgagtaacctcggaggcaaaatccgttccaatggcccaccaacaagatttattctaacaagaacatgatttctctccactgataagccatcaattataaagtccctgtggctctcagaaatctccaagatattttcttcttgagcatttagtaacatttcagatacctgatactgagcctctaacaggagaagagtgtccagatcacagcatatcacacttaataaccttagaccaaagatatgtgattgttcatagttgaataaagaacgaatcttagcttcagaattcaaaattataagtctatcaataatatcaataacacatgttgggacttcacgaagagaatattctgttttattaggaagatcttgattccttacaagctcataaatagcaggataggataacaagttcaccagtgctaaaaaagacttttgacagcttcggtcaataggatccactggagtagttctgggatgggttaccctaacatcatctcttccatattccagattggaccataattcagttataagttcattaataaaccctgacttttttagtgcaatgccacctgctgctgttgatgccactcgtgtaaccaaaactccatagccaaattttttatgcctgctgacctgtaatttttttgcatatcgattgaatataaatgtcacacattcattgatagcacctgttctttgaagaagtagtaatcctttgggggtggcagcaaaatgtagtaaatcatctaacaaattatcttcccaagccataatgttttgggattcctggcttactgaagaaacagaatcagaaccctctactggagtaggaattctttctgatagcaaacttgtctttttccatgcctttgctatagattcatgcaaattataagtgattaacacctgcaaaccttcacatgtactatatatgtgacgacacacagaaataaaagctcctttaaccacaggcaacatttctgatccagaaaatatagaaatatcttcatcgagaagttttttcgaaaactgggcaattatatgagcacctgtaggactttcttcagaagagttcatatttgctccataaaggagtaaaataagcccttcttctacagatgcaattcttgccaaaataccagctatatgaattaaagctgtctcagagcaatttggagatgcctcatttcctttcattaaattgtgaataggctgaagaagtgtctctattacaatgttgttatataagcattccactgcacattctttttgatcactgagtatccacagaacttcagtcaccatacttgcaggagagtaattctctgaatgggcagctgatgtcatctttggacaacttggtgagtaatagataagttgggtaaaaagaacaagcagatctatgagggataccaaaccttttttattcttcagcttaataggaaatagttttctgccttgtttatagatcaataatcttcctaaaaggcacagtgagtgaatgaaataaatatattgtaattcttgtcctaagtagtagaaagttttctgcttgtttctgcaatgctttgaatgtcccaaagtttcatcagctttcctagtcttacacatttcaaagtactgaacacactgttgaatggctgtagttaccagagacttatatttcgtttcaagaagtcttaatactgtagttctgctataatgtgcatgcatccactttttgaaccacacagccttggtatcaactaatgcaaaaaagtagatcggatccaaaatcttttgtgagacaacatggctttgattatgtttaactgttaacaaggacaaagtactctccacaatttcttccatatacttctctggatgacgaatccagaaagatggagcttctttctgatattcatttagaagacgaacctttttaagtaagcgagtcatattaggattagttatatctacaccagctgaaagagtaggaatatgattttccctagaaagaaagtatgactccaaatacttagctaagcttgtataaatttccttggtcatatgtaatggagaaagcaaaaatgtctgtgcacagaattttaaaatccggtcactaaacacaggatcaggatctgaaagagacacggtcagtttttcgcagagagtagtccaattttcacagttgaggacatcagatggaggagctgaacataatgtttgcaaggcttcatatctcacctctttaggttgcccaggatccaactggtctaaaatcaattgtaattttccttgacaaaatttgtaactctgattcaatgatgaatcactatcagagcaattgtctgtgcggtaactatggcttttctccttttggatttttttctgcctttcttgatttcgtgtctcatcttcttcaaacttgttaatcatagactcgaccacagctatcataatgttcttcaggtaatgcatcatttctttgtactctttagattcttgagttcttttagtgacctgctgtacaactgtatcatagccgcattcttcaccctgattccgatcagatgtgcatttttccatttcttcttcaatcatagaacccaaagtgttgcctatatgctgcctgaggtatttcacaaattcatagttgtgaaaattttcatcagtttcctccagatgtaaaagaatctcttcggcacactccagggaaggggcacccgtgattttctccttcacgctctggaacaaccgcctcagcatcgcctgcagcatcgcctggtcctcgctggagaaatgggccatcctgttggaatcaaacgtccactctcattactccaggtccgagcaaaagc

SEQ ID NO: 14400 - RNA, 4956 nt, Homo sapiens
  source 1..4956: mol_type = other RNA
gctgggattacaggcatgagccaccgcgcctggccaggactaactcttaaacatgaataagaactaaaagtaagctagatctgattctataataaccttacaaaacaacaaatttacaaaaatgaattcacaaattgagctcatacctacttaaatatatcgttatacttctcagtatttacaatatgtatattcacaaagtaaatgttgttacagacacagaaaaacatcaagcccccctgctgtgtttaaaaataaataaaacctaaatttaaaccgtgtgtctcatgatctatgtgctctgcagtctaatgttccgcatgtctctcagcagcactgttcggtagttttgttccaaaatttccatgtattcaaaataatcactcactcgaaacccatgcagtgcttcttcttttaggaaaacttgcagatcttgagtctgagtgtgctgtagaatgtcttgctgtaaatgtttgaatacagctatacagatatacacttgataatcaggaccaaggaaaacacaagtagcaatataatggcagatttctatccaatctaagtaattccaaaaacactgggttatccattgcaggcaaatctgtgatggtgcaaaaccagacatgtgaaaagctgaaaacacaagaggcaactcagccttcagtagcatttcaatataatgggtgctgcaaaaatatactggatggatgccagattctacagtgtcattaggaaggtaactagaaatatgtagccttggcaaccaaagaaaagcagaagtcagaagcctggagaattgatgaagaaattggaatgttttttctttgtctcccaacattatcatgaacagagaagatacaaaccagtcatggccagcataattcccttgcaggcagagaagagaagattttatggaagtttgctgctgtttcaggaatctctcacaatgctttaaaacccaggtaagatcattttctgcaccatcttttaagagactgaggaatttgccatacctgacagtcattttaatgccaagctgctgcacagatgaaagactttcattcttcacatttgcatcagtagctgtatactccactgaagggaagtagcattcagatgggctttcagtgagatgaagcacaaatttttcaagtaattctattaaggcctctccactgattatatcaggtttggctttcatcattttgcaaaattgtctttggcagttttctatccattcagtttgtttatcagatattttgaggcataataaaagcttgtcaagatcattgtcttgttttataccagcatttcttgtaatgtctgacagatagcagtttggcaatggatatgatgaaaacattggccaaggatatggattatcactcttttcgagtaacctcggaggcaaaatccgttccaatggcccaccaacaagatttattctaacaagaacatgatttctctccactgataagccatcaattataaagtccctgtggctctcagaaatctccaagatattttcttcttgagcatttagtaacatttcagatacctgatactgagcctctaacaggagaagagtgtccagatcacagcatatcacacttaataaccttagaccaaagatatgtgattgttcatagttgaataaagaacgaatcttagcttcagaattcaaaattataagtctatcaataatatcaataacacatgttgggacttcacgaagagaatattctgttttattaggaagatcttgattccttacaagctcataaatagcaggataggataacaagttcaccagtgctaaaaaagacttttgacagcttcggtcaataggatccactggagtagttctgggatgggttaccctaacatcatctcttccatattccagattggaccataattcagttataagttcattaataaaccctgacttttttagtgcaatgccacctgctgctgttgatgccactcgtgtaaccaaaactccatagccaaattttttatgcctgctgacctgtaatttttttgcatatcgattgaatataaatgtcacacattcattgatagcacctgttctttgaagaagtagtaatcctttgggggtggcagcaaaatgtagtaaatcatctaacaaattatcttcccaagccataatgttttgggattcctggcttactgaagaaacagaatcagaaccctctactggagtaggaattctttctgatagcaaacttgtctttttccatgcctttgctatagattcatgcaaattataagtgattaacacctgcaaaccttcacatgtactatatatgtgacgacacacagaaataaaagctcctttaaccacaggcaacatttctgatccagaaaatatagaaatatcttcatcgagaagttttttcgaaaactgggcaattatatgagcacctgtaggactttcttcagaagagttcatatttgctccataaaggagtaaaataagcccttcttctacagatgcaattcttgccaaaataccagctatatgaattaaagctgtctcagagcaatttggagatgcctcatttcctttcattaaattgtgaataggctgaagaagtgtctctattacaatgttgttatataagcattccactgcacattctttttgatcactgagtatccacagaacttcagtcaccatacttgcaggagagtaattctctgaatgggcagctgatgtcatctttggacaacttggtgagtaatagataagttgggtaaaaagaacaagcagatctatgagggataccaaaccttttttattcttcagcttaataggaaatagttttctgccttgtttatagatcaataatcttcctaaaaggcacagtgagtgaatgaaataaatatattgtaattcttgtcctaagtagtagaaagttttctgcttgtttctgcaatgctttgaatgtcccaaagtttcatcagctttcctagtcttacacatttcaaagtactgaacacactgttgaatggctgtagttaccagagacttatatttcgtttcaagaagtcttaatactgtagttctgctataatgtgcatgcatccactttttgaaccacacagccttggtatcaactaatgcaaaaaagtagatcggatccaaaatcttttgtgagacaacatggctttgattatgtttaactgttaacaaggacaaagtactctccacaatttcttccatatacttctctggatgacgaatccagaaagatggagcttctttctgatattcatttagaagacgaacctttttaagtaagcgagtcatattaggattagttatatctacaccagctgaaagagtaggaatatgattttccctagaaagaaagtatgactccaaatacttagctaagcttgtataaatttccttggtcatatgtaatggagaaagcaaaaatgtctgtgcacagaattttaaaatccggtcactaaacacaggatcaggatctgaaagagacacggtcagtttttcgcagagagtagtccaattttcacagttgaggacatcagatggaggagctgaacataatgtttgcaaggcttcatatctcacctctttaggttgcccaggatccaactggtctaaaatcaattgtaattttccttgacaaaatttgtaactctgattcaatgatgaatcactatcagagcaattgtctgtgcggtaactatggcttttctccttttggatttttttctgcctttcttgatttcgtgtctcatcttcttcaaacttgttaatcatagactcgaccacagctatcataatgttcttcaggtaatgcatcatttctttgtactctttagattcttgagttcttttagtgacctgctgtacaactgtatcatagccgcattcttcaccctgattccgatcagatgtgcatttttccatttcttcttcaatcatagaacccaaagtgttgcctatatgctgcctgaggtatttcacaaattcatagttgtgaaaattttcatcagtttcctccagatgtaaaagaatctcttcggcacactccagggaaggggcacccgtgattttctccttcacgctctggaacaaccgcctcagcatcgcctgcagcatcgcctggtcctcgctggagaaatgggccatccttactttggggaagcaggggtccgcgaggtctcgcctctggtactcttagttgctagccttcagtaccagcagacctcaggctctcccgactaacaacaaaagagacatcaggaatgatctgatgggaggacccgacgacggaacgccacgatgcgcgtgacgtcagctcgctgatgtggcttccttggtgggagggagtgcaactggtgtcctgggggcgcccagagaatgttcgggtgagccactctccttcgccgccgcgttgtaggtgggagggaagagagtacgaagagaaagtgatcaataaaagaaagatagtaaaagtgaaactgaaagtagcctgacgagcctcagttgaagagtgaatggtattgaaaagttgcagtgttgttttcctctaacggctaacacctattgagctcctacgccctaccaaacactttccttaccaagcaccctgctaggagctatgaagaactccctcactaagtaacagagagaaaaataaattaacgattacaatacagtgcaattaaatgtcatgctagaaaaaaaagatatgccaagtcggtgctgtggagacccagaattagtttcaacccaatagaggagttgaggaaagaagcaaagagagtaaactggacatgcaaagaataggggcctcagagtgtaggatatactggcacttgaggtaatcgggttagaaagaggagatgaggaagctaaagaagtaaattggtcacatctggaagggtctaatcttt

SEQ ID NO: 14401 - RNA, 4302 nt, Homo sapiens
  source 1..4302: mol_type = other RNA
gctgggattacaggcatgagccaccgcgcctggccaggactaactcttaaacatgaataagaactaaaagtaagctagatctgattctataataaccttacaaaacaacaaatttacaaaaatgaattcacaaattgagctcatacctacttaaatatatcgttatacttctcagtatttacaatatgtatattcacaaagtaaatgttgttacagacacagaaaaacatcaagcccccctgctgtgtttaaaaataaataaaacctaaatttaaaccgtgtgtctcatgatctatgtgctctgcagtctaatgttccgcatgtctctcagcagcactgttcggtagttttgttccaaaatttccatgtattcaaaataatcactcactcgaaacccatgcagtgcttcttcttttaggaaaacttgcagatcttgagtctgagtgtgctgtagaatgtcttgctgtaaatgtttgaatacagctatacagatatacacttgataatcaggaccaaggaaaacacaagtagcaatataatggcagatttctatccaatctaagtaattccaaaaacactgggttatccattgcaggcaaatctgtgatggtgcaaaaccagacatgtgaaaagctgaaaacacaagaggcaactcagccttcagtagcatttcaatataatgggtgctgcaaaaatatactggatggatgccagattctacagtgtcattaggaaggtaactagaaatatgtagccttggcaaccaaagaaaagcagaagtcagaagcctggagaattgatgaagaaattggaatgttttttctttgtctcccaacattatcatgaacagagaagatacaaaccagtcatggccagcataattcccttgcaggcagagaagagaagattttatggaagtttgctgctgtttcaggaatctctcacaatgctttaaaacccaggtaagatcattttctgcaccatcttttaagagactgaggaatttgccatacctgacagtcattttaatgccaagctgctgcacagatgaaagactttcattcttcacatttgcatcagtagctgtatactccactgaagggaagtagcattcagatgggctttcagtgagatgaagcacaaatttttcaagtaattctattaaggcctctccactgattatatcaggtttggctttcatcattttgcaaaattgtctttggcagttttctatccattcagtttgtttatcagatattttgaggcataataaaagcttgtcaagatcattgtcttgttttataccagcatttcttgtaatgtctgacagatagcagtttggcaatggatatgatgaaaacattggccaaggatatggattatcactcttttcgagtaacctcggaggcaaaatccgttccaatggcccaccaacaagatttattctaacaagaacatgatttctctccactgataagccatcaattataaagtccctgtggctctcagaaatctccaagatattttcttcttgagcatttagtaacatttcagatacctgatactgagcctctaacaggagaagagtgtccagatcacagcatatcacacttaataaccttagaccaaagatatgtgattgttcatagttgaataaagaacgaatcttagcttcagaattcaaaattataagtctatcaataatatcaataacacatgttgggacttcacgaagagaatattctgttttattaggaagatcttgattccttacaagctcataaatagcaggataggataacaagttcaccagtgctaaaaaagacttttgacagcttcggtcaataggatccactggagtagttctgggatgggttaccctaacatcatctcttccatattccagattggaccataattcagttataagttcattaataaaccctgacttttttagtgcaatgccacctgctgctgttgatgccactcgtgtaaccaaaactccatagccaaattttttatgcctgctgacctgtaatttttttgcatatcgattgaatataaatgtcacacattcattgatagcacctgttctttgaagaagtagtaatcctttgggggtggcagcaaaatgtagtaaatcatctaacaaattatcttcccaagccataatgttttgggattcctggcttactgaagaaacagaatcagaaccctctactggagtaggaattctttctgatagcaaacttgtctttttccatgcctttgctatagattcatgcaaattataagtgattaacacctgcaaaccttcacatgtactatatatgtgacgacacacagaaataaaagctcctttaaccacaggcaacatttctgatccagaaaatatagaaatatcttcatcgagaagttttttcgaaaactgggcaattatatgagcacctgtaggactttcttcagaagagttcatatttgctccataaaggagtaaaataagcccttcttctacagatgcaattcttgccaaaataccagctatatgaattaaagctgtctcagagcaatttggagatgcctcatttcctttcattaaattgtgaataggctgaagaagtgtctctattacaatgttgttatataagcattccactgcacattctttttgatcactgagtatccacagaacttcagtcaccatacttgcaggagagtaattctctgaatgggcagctgatgtcatctttggacaacttggtgagtaatagataagttgggtaaaaagaacaagcagatctatgagggataccaaaccttttttattcttcagcttaataggaaatagttttctgccttgtttatagatcaataatcttcctaaaaggcacagtgagtgaatgaaataaatatattgtaattcttgtcctaagtagtagaaagttttctgcttgtttctgcaatgctttgaatgtcccaaagtttcatcagctttcctagtcttacacatttcaaagtactgaacacactgttgaatggctgtagttaccagagacttatatttcgtttcaagaagtcttaatactgtagttctgctataatgtgcatgcatccactttttgaaccacacagccttggtatcaactaatgcaaaaaagtagatcggatccaaaatcttttgtgagacaacatggctttgattatgtttaactgttaacaaggacaaagtactctccacaatttcttccatatacttctctggatgacgaatccagaaagatggagcttctttctgatattcatttagaagacgaacctttttaagtaagcgagtcatattaggattagttatatctacaccagctgaaagagtaggaatatgattttccctagaaagaaagtatgactccaaatacttagctaagcttgtataaatttccttggtcatatgtaatggagaaagcaaaaatgtctgtgcacagaattttaaaatccggtcactaaacacaggatcaggatctgaaagagacacggtcagtttttcgcagagagtagtccaattttcacagttgaggacatcagatggaggagctgaacataatgtttgcaaggcttcatatctcacctctttaggttgcccaggatccaactggtctaaaatcaattgtaattttccttgacaaaatttgtaactctgattcaatgatgaatcactatcagagcaattgtctgtgcggtaactatggcttttctccttttggatttttttctgcctttcttgatttcgtgtctcatcttcttcaaacttgttaatcatagactcgaccacagctatcataatgttcttcaggtaatgcatcatttctttgtactctttagattcttgagttcttttagtgacctgctgtacaactgtatcatagccgcattcttcaccctgattccgatcagatgtgcatttttccatttcttcttcaatcatagaacccaaagtgttgcctatatgctgcctgaggtatttcacaaattcatagttgtgaaaattttcatcagtttcctccagatgtaaaagaatctcttcggcacactccagggaaggggcacccgtgattttctccttcacgctctggaacaaccgcctcagcatcgcctgcagcatcgcctggtcctcgctggagaaatgggccatctttggggaagcaggggtccgcgaggtctcgcctctggtactcttagttgctagccttcagtaccagcagacctcaggctctcccgactaacaacaaaagagacatcaggaat

SEQ ID NO: 14402 - RNA, 4116 nt, Homo sapiens
  source 1..4116: mol_type = other RNA
gctgggattacaggcatgagccaccgcgcctggccaggactaactcttaaacatgaataagaactaaaagtaagctagatctgattctataataaccttacaaaacaacaaatttacaaaaatgaattcacaaattgagctcatacctacttaaatatatcgttatacttctcagtatttacaatatgtatattcacaaagtaaatgttgttacagacacagaaaaacatcaagcccccctgctgtgtttaaaaataaataaaacctaaatttaaaccgtgtgtctcatgatctatgtgctctgcagtctaatgttccgcatgtctctcagcagcactgttcggtagttttgttccaaaatttccatgtattcaaaataatcactcactcgaaacccatgcagtgcttcttcttttaggaaaacttgcagatcttgagtctgagtgtgctgtagaatgtcttgctgtaaatgtttgaatacagctatacagatatacacttgataatcaggaccaaggaaaacacaagtagcaatataatggcagatttctatccaatctaagtaattccaaaaacactgggttatccattgcaggcaaatctgtgatggtgcaaaaccagacatgtgaaaagctgaaaacacaagaggcaactcagccttcagtagcatttcaatataatgggtgctgcaaaaatatactggatggatgccagattctacagtgtcattaggaaggtaactagaaatatgtagccttggcaaccaaagaaaagcagaagtcagaagcctggagaattgatgaagaaattggaatgttttttctttgtctcccaacattatcatgaacagagaagatacaaaccagtcatggccagcataattcccttgcaggcagagaagagaagattttatggaagtttgctgctgtttcaggaatctctcacaatgctttaaaacccaggtaagatcattttctgcaccatcttttaagagactgaggaatttgccatacctgacagtcattttaatgccaagctgctgcacagatgaaagactttcattcttcacatttgcatcagtagctgtatactccactgaagggaagtagcattcagatgggctttcagtgagatgaagcacaaatttttcaagtaattctattaaggcctctccactgattatatcaggtttggctttcatcattttgcaaaattgtctttggcagttttctatccattcagtttgtttatcagatattttgaggcataataaaagcttgtcaagatcattgtcttgttttataccagcatttcttgtaatgtctgacagatagcagtttggcaatggatatgatgaaaacattggccaaggatatggattatcactcttttcgagtaacctcggaggcaaaatccgttccaatggcccaccaacaagatttattctaacaagaacatgatttctctccactgataagccatcaattataaagtcccttagaccaaagatatgtgattgttcatagttgaataaagaacgaatcttagcttcagaattcaaaattataagtctatcaataatatcaataacacatgttgggacttcacgaagagaatattctgttttattaggaagatcttgattccttacaagctcataaatagcaggataggataacaagttcaccagtgctaaaaaagacttttgacagcttcggtcaataggatccactggagtagttctgggatgggttaccctaacatcatctcttccatattccagattggaccataattcagttataagttcattaataaaccctgacttttttagtgcaatgccacctgctgctgttgatgccactcgtgtaaccaaaactccatagccaaattttttatgcctgctgacctgtaatttttttgcatatcgattgaatataaatgtcacacattcattgatagcacctgttctttgaagaagtagtaatcctttgggggtggcagcaaaatgtagtaaatcatctaacaaattatcttcccaagccataatgttttgggattcctggcttactgaagaaacagaatcagaaccctctactggagtaggaattctttctgatagcaaacttgtctttttccatgcctttgctatagattcatgcaaattataagtgattaacacctgcaaaccttcacatgtactatatatgtgacgacacacagaaataaaagctcctttaaccacaggcaacatttctgatccagaaaatatagaaatatcttcatcgagaagttttttcgaaaactgggcaattatatgagcacctgtaggactttcttcagaagagttcatatttgctccataaaggagtaaaataagcccttcttctacagatgcaattcttgccaaaataccagctatatgaattaaagctgtctcagagcaatttggagatgcctcatttcctttcattaaattgtgaataggctgaagaagtgtctctattacaatgttgttatataagcattccactgcacattctttttgatcactgagtatccacagaacttcagtcaccatacttgcaggagagtaattctctgaatgggcagctgatgtcatctttggacaacttggtgagtaatagataagttgggtaaaaagaacaagcagatctatgagggataccaaaccttttttattcttcagcttaataggaaatagttttctgccttgtttatagatcaataatcttcctaaaaggcacagtgagtgaatgaaataaatatattgtaattcttgtcctaagtagtagaaagttttctgcttgtttctgcaatgctttgaatgtcccaaagtttcatcagctttcctagtcttacacatttcaaagtactgaacacactgttgaatggctgtagttaccagagacttatatttcgtttcaagaagtcttaatactgtagttctgctataatgtgcatgcatccactttttgaaccacacagccttggtatcaactaatgcaaaaaagtagatcggatccaaaatcttttgtgagacaacatggctttgattatgtttaactgttaacaaggacaaagtactctccacaatttcttccatatacttctctggatgacgaatccagaaagatggagcttctttctgatattcatttagaagacgaacctttttaagtaagcgagtcatattaggattagttatatctacaccagctgaaagagtaggaatatgattttccctagaaagaaagtatgactccaaatacttagctaagcttgtataaatttccttggtcatatgtaatggagaaagcaaaaatgtctgtgcacagaattttaaaatccggtcactaaacacaggatcaggatctgaaagagacacggtcagtttttcgcagagagtagtccaattttcacagttgaggacatcagatggaggagctgaacataatgtttgcaaggcttcatatctcacctctttaggttgcccaggatccaactggtctaaaatcaattgtaattttccttgacaaaatttgtaactctgattcaatgatgaatcactatcagagcaattgtctgtgcggtaactatggcttttctccttttggatttttttctgcctttcttgatttcgtgtctcatcttcttcaaacttgttaatcatagactcgaccacagctatcataatgttcttcaggtaatgcatcatttctttgtactctttagattcttgagttcttttagtgacctgctgtacaactgtatcatagccgcattcttcaccctgattccgatcagatgtgcatttttccatttcttcttcaatcatagaacccaaagtgttgcctatatgctgcctgaggtatttcacaaattcatagttgtgaaaattttcatcagtttcctccagatgtaaaagaatctcttcggcacactccagggaaggggcacccgtgattttctccttcacgctctggaacaaccgcctcagcatcgcctgcagcatcgcctggtcctcgctggagaaatgggccatcctgttggaatcaaacgtccactctcattactccaggtccgagcaaaagc

SEQ ID NO: 14403 - RNA, 4184 nt, Homo sapiens
  source 1..4184: mol_type = other RNA
gctgggattacaggcatgagccaccgcgcctggccaggactaactcttaaacatgaataagaactaaaagtaagctagatctgattctataataaccttacaaaacaacaaatttacaaaaatgaattcacaaattgagctcatacctacttaaatatatcgttatacttctcagtatttacaatatgtatattcacaaagtaaatgttgttacagacacagaaaaacatcaagcccccctgctgtgtttaaaaataaataaaacctaaatttaaaccgtgtgtctcatgatctatgtgctctgcagtctaatgttccgcatgtctctcagcagcactgttcggtagttttgttccaaaatttccatgtattcaaaataatcactcactcgaaacccatgcagtgcttcttcttttaggaaaacttgcagatcttgagtctgagtgtgctgtagaatgtcttgctgtaaatgtttgaatacagctatacagatatacacttgataatcaggaccaaggaaaacacaagtagcaatataatggcagatttctatccaatctaagtaattccaaaaacactgggttatccattgcaggcaaatctgtgatggtgcaaaaccagacatgtgaaaagctgaaaacacaagaggcaactcagccttcagtagcatttcaatataatgggtgctgcaaaaatatactggatggatgccagattctacagtgtcattaggaaggtaactagaaatatgtagccttggcaaccaaagaaaagcagaagtcagaagcctggagaattgatgaagaaattggaatgttttttctttgtctcccaacattatcatgaacagagaagatacaaaccagtcatggccagcataattcccttgcaggcagagaagagaagattttatggaagtttgctgctgtttcaggaatctctcacaatgctttaaaacccaggtaagatcattttctgcaccatcttttaagagactgaggaatttgccatacctgacagtcattttaatgccaagctgctgcacagatgaaagactttcattcttcacatttgcatcagtagctgtatactccactgaagggaagtagcattcagatgggctttcagtgagatgaagcacaaatttttcaagtaattctattaaggcctctccactgattatatcaggtttggctttcatcattttgcaaaattgtctttggcagttttctatccattcagtttgtttatcagatattttgaggcataataaaagcttgtcaagatcattgtcttgttttataccagcatttcttgtaatgtctgacagatagcagtttggcaatggatatgatgaaaacattggccaaggatatggattatcactcttttcgagtaacctcggaggcaaaatccgttccaatggcccaccaacaagatttattctaacaagaacatgatttctctccactgataagccatcaattataaagtcccttagaccaaagatatgtgattgttcatagttgaataaagaacgaatcttagcttcagaattcaaaattataagtctatcaataatatcaataacacatgttgggacttcacgaagagaatattctgttttattaggaagatcttgattccttacaagctcataaatagcaggataggataacaagttcaccagtgctaaaaaagacttttgacagcttcggtcaataggatccactggagtagttctgggatgggttaccctaacatcatctcttccatattccagattggaccataattcagttataagttcattaataaaccctgacttttttagtgcaatgccacctgctgctgttgatgccactcgtgtaaccaaaactccatagccaaattttttatgcctgctgacctgtaatttttttgcatatcgattgaatataaatgtcacacattcattgatagcacctgttctttgaagaagtagtaatcctttgggggtggcagcaaaatgtagtaaatcatctaacaaattatcttcccaagccataatgttttgggattcctggcttactgaagaaacagaatcagaaccctctactggagtaggaattctttctgatagcaaacttgtctttttccatgcctttgctatagattcatgcaaattataagtgattaacacctgcaaaccttcacatgtactatatatgtgacgacacacagaaataaaagctcctttaaccacaggcaacatttctgatccagaaaatatagaaatatcttcatcgagaagttttttcgaaaactgggcaattatatgagcacctgtaggactttcttcagaagagttcatatttgctccataaaggagtaaaataagcccttcttctacagatgcaattcttgccaaaataccagctatatgaattaaagctgtctcagagcaatttggagatgcctcatttcctttcattaaattgtgaataggctgaagaagtgtctctattacaatgttgttatataagcattccactgcacattctttttgatcactgagtatccacagaacttcagtcaccatacttgcaggagagtaattctctgaatgggcagctgatgtcatctttggacaacttggtgagtaatagataagttgggtaaaaagaacaagcagatctatgagggataccaaaccttttttattcttcagcttaataggaaatagttttctgccttgtttatagatcaataatcttcctaaaaggcacagtgagtgaatgaaataaatatattgtaattcttgtcctaagtagtagaaagttttctgcttgtttctgcaatgctttgaatgtcccaaagtttcatcagctttcctagtcttacacatttcaaagtactgaacacactgttgaatggctgtagttaccagagacttatatttcgtttcaagaagtcttaatactgtagttctgctataatgtgcatgcatccactttttgaaccacacagccttggtatcaactaatgcaaaaaagtagatcggatccaaaatcttttgtgagacaacatggctttgattatgtttaactgttaacaaggacaaagtactctccacaatttcttccatatacttctctggatgacgaatccagaaagatggagcttctttctgatattcatttagaagacgaacctttttaagtaagcgagtcatattaggattagttatatctacaccagctgaaagagtaggaatatgattttccctagaaagaaagtatgactccaaatacttagctaagcttgtataaatttccttggtcatatgtaatggagaaagcaaaaatgtctgtgcacagaattttaaaatccggtcactaaacacaggatcaggatctgaaagagacacggtcagtttttcgcagagagtagtccaattttcacagttgaggacatcagatggaggagctgaacataatgtttgcaaggcttcatatctcacctctttaggttgcccaggatccaactggtctaaaatcaattgtaattttccttgacaaaatttgtaactctgattcaatgatgaatcactatcagagcaattgtctgtgcggtaactatggcttttctccttttggatttttttctgcctttcttgatttcgtgtctcatcttcttcaaacttgttaatcatagactcgaccacagctatcataatgttcttcaggtaatgcatcatttctttgtactctttagattcttgagttcttttagtgacctgctgtacaactgtatcatagccgcattcttcaccctgattccgatcagatgtgcatttttccatttcttcttcaatcatagaacccaaagtgttgcctatatgctgcctgaggtatttcacaaattcatagttgtgaaaattttcatcagtttcctccagatgtaaaagaatctcttcggcacactccagggaaggggcacccgtgattttctccttcacgctctggaacaaccgcctcagcatcgcctgcagcatcgcctggtcctcgctggagaaatgggccatctttggggaagcaggggtccgcgaggtctcgcctctggtactcttagttgctagccttcagtaccagcagacctcaggctctcccgactaacaacaaaagagacatcaggaatgatct

SEQ ID NO: 14404 - RNA, 4318 nt, Homo sapiens
  source 1..4318: mol_type = other RNA
gctgggattacaggcatgagccaccgcgcctggccaggactaactcttaaacatgaataagaactaaaagtaagctagatctgattctataataaccttacaaaacaacaaatttacaaaaatgaattcacaaattgagctcatacctacttaaatatatcgttatacttctcagtatttacaatatgtatattcacaaagtaaatgttgttacagacacagaaaaacatcaagcccccctgctgtgtttaaaaataaataaaacctaaatttaaaccgtgtgtctcatgatctatgtgctctgcagtctaatgttccgcatgtctctcagcagcactgttcggtagttttgttccaaaatttccatgtattcaaaataatcactcactcgaaacccatgcagtgcttcttcttttaggaaaacttgcagatcttgagtctgagtgtgctgtagaatgtcttgctgtaaatgtttgaatacagctatacagatatacacttgataatcaggaccaaggaaaacacaagtagcaatataatggcagatttctatccaatctaagtaattccaaaaacactgggttatccattgcaggcaaatctgtgatggtgcaaaaccagacatgtgaaaagctgaaaacacaagaggcaactcagccttcagtagcatttcaatataatgggtgctgcaaaaatatactggatggatgccagattctacagtgtcattaggaaggtaactagaaatatgtagccttggcaaccaaagaaaagcagaagtcagaagcctggagaattgatgaagaaattggaatgttttttctttgtctcccaacattatcatgaacagagaagatacaaaccagtcatggccagcataattcccttgcaggcagagaagagaagattttatggaagtttgctgctgtttcaggaatctctcacaatgctttaaaacccaggtaagatcattttctgcaccatcttttaagagactgaggaatttgccatacctgacagtcattttaatgccaagctgctgcacagatgaaagactttcattcttcacatttgcatcagtagctgtatactccactgaagggaagtagcattcagatgggctttcagtgagatgaagcacaaatttttcaagtaattctattaaggcctctccactgattatatcaggtttggctttcatcattttgcaaaattgtctttggcagttttctatccattcagtttgtttatcagatattttgaggcataataaaagcttgtcaagatcattgttcactgaacgctgcatagctccagagacacagaatatggtattcttgttctttggccccatctcttgttttataccagcatttcttgtaatgtctgacagatagcagtttggcaatggatatgatgaaaacattggccaaggatatggattatcactcttttcgagtaacctcggaggcaaaatccgttccaatggcccaccaacaagatttattctaacaagaacatgatttctctccactgataagccatcaattataaagtccctgtggctctcagaaatctccaagatattttcttcttgagcatttagtaacatttcagatacctgatactgagcctctaacaggagaagagtgtccagatcacagcatatcacacttaataaccttagaccaaagatatgtgattgttcatagttgaataaagaacgaatcttagcttcagaattcaaaattataagtctatcaataatatcaataacacatgttgggacttcacgaagagaatattctgttttattaggaagatcttgattccttacaagctcataaatagcaggataggataacaagttcaccagtgctaaaaaagacttttgacagcttcggtcaataggatccactggagtagttctgggatgggttaccctaacatcatctcttccatattccagattggaccataattcagttataagttcattaataaaccctgacttttttagtgcaatgccacctgctgctgttgatgccactcgtgtaaccaaaactccatagccaaattttttatgcctgctgacctgtaatttttttgcatatcgattgaatataaatgtcacacattcattgatagcacctgttctttgaagaagtagtaatcctttgggggtggcagcaaaatgtagtaaatcatctaacaaattatcttcccaagccataatgttttgggattcctggcttactgaagaaacagaatcagaaccctctactggagtaggaattctttctgatagcaaacttgtctttttccatgcctttgctatagattcatgcaaattataagtgattaacacctgcaaaccttcacatgtactatatatgtgacgacacacagaaataaaagctcctttaaccacaggcaacatttctgatccagaaaatatagaaatatcttcatcgagaagttttttcgaaaactgggcaattatatgagcacctgtaggactttcttcagaagagttcatatttgctccataaaggagtaaaataagcccttcttctacagatgcaattcttgccaaaataccagctatatgaattaaagctgtctcagagcaatttggagatgcctcatttcctttcattaaattgtgaataggctgaagaagtgtctctattacaatgttgttatataagcattccactgcacattctttttgatcactgagtatccacagaacttcagtcaccatacttgcaggagagtaattctctgaatgggcagctgatgtcatctttggacaacttggtgagtaatagataagttgggtaaaaagaacaagcagatctatgagggataccaaaccttttttattcttcagcttaataggaaatagttttctgccttgtttatagatcaataatcttcctaaaaggcacagtgagtgaatgaaataaatatattgtaattcttgtcctaagtagtagaaagttttctgcttgtttctgcaatgctttgaatgtcccaaagtttcatcagctttcctagtcttacacatttcaaagtactgaacacactgttgaatggctgtagttaccagagacttatatttcgtttcaagaagtcttaatactgtagttctgctataatgtgcatgcatccactttttgaaccacacagccttggtatcaactaatgcaaaaaagtagatcggatccaaaatcttttgtgagacaacatggctttgattatgtttaactgttaacaaggacaaagtactctccacaatttcttccatatacttctctggatgacgaatccagaaagatggagcttctttctgatattcatttagaagacgaacctttttaagtaagcgagtcatattaggattagttatatctacaccagctgaaagagtaggaatatgattttccctagaaagaaagtatgactccaaatacttagctaagcttgtataaatttccttggtcatatgtaatggagaaagcaaaaatgtctgtgcacagaattttaaaatccggtcactaaacacaggatcaggatctgaaagagacacggtcagtttttcgcagagagtagtccaattttcacagttgaggacatcagatggaggagctgaacataatgtttgcaaggcttcatatctcacctctttaggttgcccaggatccaactggtctaaaatcaattgtaattttccttgacaaaatttgtaactctgattcaatgatgaatcactatcagagcaattgtctgtgcggtaactatggcttttctccttttggatttttttctgcctttcttgatttcgtgtctcatcttcttcaaacttgttaatcatagactcgaccacagctatcataatgttcttcaggtaatgcatcatttctttgtacctttaaattcaaggtagttctttagattcttgagttcttttagtgacctgctgtacaactgtatcatagccgcattcttcaccctgattccgatcagatgtgcatttttccatttcttcttcaatcatagaacccaaagtgttgcctatatgctgcctgaggtatttcacaaattcatagttgtgaaaattttcatcagtttcctccagatgtaaaagaatctcttcggcacactccagggaaggggcacccgtgattttctccttcacgctctggaacaaccgcctcagcatcgcctgcagcatcgcctggtcctcgctggagaaatgggccatcctgttggaatcaaacgtccactctcattactccaggtccgagcaaaa

SEQ ID NO: 14405 - RNA, 4320 nt, Homo sapiens
  source 1..4320: mol_type = other RNA
gctgggattacaggcatgagccaccgcgcctggccaggactaactcttaaacatgaataagaactaaaagtaagctagatctgattctataataaccttacaaaacaacaaatttacaaaaatgaattcacaaattgagctcatacctacttaaatatatcgttatacttctcagtatttacaatatgtatattcacaaagtaaatgttgttacagacacagaaaaacatcaagcccccctgctgtgtttaaaaataaataaaacctaaatttaaaccgtgtgtctcatgatctatgtgctctgcagtctaatgttccgcatgtctctcagcagcactgttcggtagttttgttccaaaatttccatgtattcaaaataatcactcactcgaaacccatgcagtgcttcttcttttaggaaaacttgcagatcttgagtctgagtgtgctgtagaatgtcttgctgtaaatgtttgaatacagctatacagatatacacttgataatcaggaccaaggaaaacacaagtagcaatataatggcagatttctatccaatctaagtaattccaaaaacactgggttatccattgcaggcaaatctgtgatggtgcaaaaccagacatgtgaaaagctgaaaacacaagaggcaactcagccttcagtagcatttcaatataatgggtgctgcaaaaatatactggatggatgccagattctacagtgtcattaggaaggtaactagaaatatgtagccttggcaaccaaagaaaagcagaagtcagaagcctggagaattgatgaagaaattggaatgttttttctttgtctcccaacattatcatgaacagagaagatacaaaccagtcatggccagcataattcccttgcaggcagagaagagaagattttatggaagtttgctgctgtttcaggaatctctcacaatgctttaaaacccaggtaagatcattttctgcaccatcttttaagagactgaggaatttgccatacctgacagtcattttaatgccaagctgctgcacagatgaaagactttcattcttcacatttgcatcagtagctgtatactccactgaagggaagtagcattcagatgggctttcagtgagatgaagcacaaatttttcaagtaattctattaaggcctctccactgattatatcaggtttggctttcatcattttgcaaaattgtctttggcagttttctatccattcagtttgtttatcagatattttgaggcataataaaagcttgtcaagatcattgttcactgaacgctgcatagctccagagacacagaatatggtattcttgttctttggccccatctcttgttttataccagcatttcttgtaatgtctgacagatagcagtttggcaatggatatgatgaaaacattggccaaggatatggattatcactcttttcgagtaacctcggaggcaaaatccgttccaatggcccaccaacaagatttattctaacaagaacatgatttctctccactgataagccatcaattataaagtccctgtggctctcagaaatctccaagatattttcttcttgagcatttagtaacatttcagatacctgatactgagcctctaacaggagaagagtgtccagatcacagcatatcacacttaataaccttagaccaaagatatgtgattgttcatagttgaataaagaacgaatcttagcttcagaattcaaaattataagtctatcaataatatcaataacacatgttgggacttcacgaagagaatattctgttttattaggaagatcttgattccttacaagctcataaatagcaggataggataacaagttcaccagtgctaaaaaagacttttgacagcttcggtcaataggatccactggagtagttctgggatgggttaccctaacatcatctcttccatattccagattggaccataattcagttataagttcattaataaaccctgacttttttagtgcaatgccacctgctgctgttgatgccactcgtgtaaccaaaactccatagccaaattttttatgcctgctgacctgtaatttttttgcatatcgattgaatataaatgtcacacattcattgatagcacctgttctttgaagaagtagtaatcctttgggggtggcagcaaaatgtagtaaatcatctaacaaattatcttcccaagccataatgttttgggattcctggcttactgaagaaacagaatcagaaccctctactggagtaggaattctttctgatagcaaacttgtctttttccatgcctttgctatagattcatgcaaattataagtgattaacacctgcaaaccttcacatgtactatatatgtgacgacacacagaaataaaagctcctttaaccacaggcaacatttctgatccagaaaatatagaaatatcttcatcgagaagttttttcgaaaactgggcaattatatgagcacctgtaggactttcttcagaagagttcatatttgctccataaaggagtaaaataagcccttcttctacagatgcaattcttgccaaaataccagctatatgaattaaagctgtctcagagcaatttggagatgcctcatttcctttcattaaattgtgaataggctgaagaagtgtctctattacaatgttgttatataagcattccactgcacattctttttgatcactgagtatccacagaacttcagtcaccatacttgcaggagagtaattctctgaatgggcagctgatgtcatctttggacaacttggtgagtaatagataagttgggtaaaaagaacaagcagatctatgagggataccaaaccttttttattcttcagcttaataggaaatagttttctgccttgtttatagatcaataatcttcctaaaaggcacagtgagtgaatgaaataaatatattgtaattcttgtcctaagtagtagaaagttttctgcttgtttctgcaatgctttgaatgtcccaaagtttcatcagctttcctagtcttacacatttcaaagtactgaacacactgttgaatggctgtagttaccagagacttatatttcgtttcaagaagtcttaatactgtagttctgctataatgtgcatgcatccactttttgaaccacacagccttggtatcaactaatgcaaaaaagtagatcggatccaaaatcttttgtgagacaacatggctttgattatgtttaactgttaacaaggacaaagtactctccacaatttcttccatatacttctctggatgacgaatccagaaagatggagcttctttctgatattcatttagaagacgaacctttttaagtaagcgagtcatattaggattagttatatctacaccagctgaaagagtaggaatatgattttccctagaaagaaagtatgactccaaatacttagctaagcttgtataaatttccttggtcatatgtaatggagaaagcaaaaatgtctgtgcacagaattttaaaatccggtcactaaacacaggatcaggatctgaaagagacacggtcagtttttcgcagagagtagtccaattttcacagttgaggacatcagatggaggagctgaacataatgtttgcaaggcttcatatctcacctctttaggttgcccaggatccaactggtctaaaatcaattgtaattttccttgacaaaatttgtaactctgattcaatgatgaatcactatcagagcaattgtctgtgcggtaactatggcttttctccttttggatttttttctgcctttcttgatttcgtgtctcatcttcttcaaacttgttaatcatagactcgaccacagctatcataatgttcttcaggtaatgcatcatttctttgtactctttagattcttgagttcttttagtgacctgctgtacaactgtatcatagccgcattcttcaccctgattccgatcagatgtgcatttttccatttcttcttcaatcatagaacccaaagtgttgcctatatgctgcctgaggtatttcacaaattcatagttgtgaaaattttcatcagtttcctccagatgtaaaagaatctcttcggcacactccagggaaggggcacccgtgattttctccttcacgctctggaacaaccgcctcagcatcgcctgcagcatcgcctggtcctcgctggagaaatgggccatcctgttggaatcaaacgtccactctcattactccaggtccgagcaaaagccgcgcactgcgcacgcgc

SEQ ID NO: 14406 - RNA, 5025 nt, Homo sapiens
  source 1..5025: mol_type = other RNA
gctgggattacaggcatgagccaccgcgcctggccaggactaactcttaaacatgaataagaactaaaagtaagctagatctgattctataataaccttacaaaacaacaaatttacaaaaatgaattcacaaattgagctcatacctacttaaatatatcgttatacttctcagtatttacaatatgtatattcacaaagtaaatgttgttacagacacagaaaaacatcaagcccccctgctgtgtttaaaaataaataaaacctaaatttaaaccgtgtgtctcatgatctatgtgctctgcagtctaatgttccgcatgtctctcagcagcactgttcggtagttttgttccaaaatttccatgtattcaaaataatcactcactcgaaacccatgcagtgcttcttcttttaggaaaacttgcagatcttgagtctgagtgtgctgtagaatgtcttgctgtaaatgtttgaatacagctatacagatatacacttgataatcaggaccaaggaaaacacaagtagcaatataatggcagatttctatccaatctaagtaattccaaaaacactgggttatccattgcaggcaaatctgtgatggtgcaaaaccagacatgtgaaaagctgaaaacacaagaggcaactcagccttcagtagcatttcaatataatgggtgctgcaaaaatatactggatggatgccagattctacagtgtcattaggaaggtaactagaaatatgtagccttggcaaccaaagaaaagcagaagtcagaagcctggagaattgatgaagaaattggaatgttttttctttgtctcccaacattatcatgaacagagaagatacaaaccagtcatggccagcataattcccttgcaggcagagaagagaagattttatggaagtttgctgctgtttcaggaatctctcacaatgctttaaaacccaggtaagatcattttctgcaccatcttttaagagactgaggaatttgccatacctgacagtcattttaatgccaagctgctgcacagatgaaagactttcattcttcacatttgcatcagtagctgtatactccactgaagggaagtagcattcagatgggctttcagtgagatgaagcacaaatttttcaagtaattctattaaggcctctccactgattatatcaggtttggctttcatcattttgcaaaattgtctttggcagttttctatccattcagtttgtttatcagatattttgaggcataataaaagcttgtcaagatcattgttcactgaacgctgcatagctccagagacacagaatatggtattcttgttctttggccccatctcttgttttataccagcatttcttgtaatgtctgacagatagcagtttggcaatggatatgatgaaaacattggccaaggatatggattatcactcttttcgagtaacctcggaggcaaaatccgttccaatggcccaccaacaagatttattctaacaagaacatgatttctctccactgataagccatcaattataaagtccctgtggctctcagaaatctccaagatattttcttcttgagcatttagtaacatttcagatacctgatactgagcctctaacaggagaagagtgtccagatcacagcatatcacacttaataaccttagaccaaagatatgtgattgttcatagttgaataaagaacgaatcttagcttcagaattcaaaattataagtctatcaataatatcaataacacatgttgggacttcacgaagagaatattctgttttattaggaagatcttgattccttacaagctcataaatagcaggataggataacaagttcaccagtgctaaaaaagacttttgacagcttcggtcaataggatccactggagtagttctgggatgggttaccctaacatcatctcttccatattccagattggaccataattcagttataagttcattaataaaccctgacttttttagtgcaatgccacctgctgctgttgatgccactcgtgtaaccaaaactccatagccaaattttttatgcctgctgacctgtaatttttttgcatatcgattgaatataaatgtcacacattcattgatagcacctgttctttgaagaagtagtaatcctttgggggtggcagcaaaatgtagtaaatcatctaacaaattatcttcccaagccataatgttttgggattcctggcttactgaagaaacagaatcagaaccctctactggagtaggaattctttctgatagcaaacttgtctttttccatgcctttgctatagattcatgcaaattataagtgattaacacctgcaaaccttcacatgtactatatatgtgacgacacacagaaataaaagctcctttaaccacaggcaacatttctgatccagaaaatatagaaatatcttcatcgagaagttttttcgaaaactgggcaattatatgagcacctgtaggactttcttcagaagagttcatatttgctccataaaggagtaaaataagcccttcttctacagatgcaattcttgccaaaataccagctatatgaattaaagctgtctcagagcaatttggagatgcctcatttcctttcattaaattgtgaataggctgaagaagtgtctctattacaatgttgttatataagcattccactgcacattctttttgatcactgagtatccacagaacttcagtcaccatacttgcaggagagtaattctctgaatgggcagctgatgtcatctttggacaacttggtgagtaatagataagttgggtaaaaagaacaagcagatctatgagggataccaaaccttttttattcttcagcttaataggaaatagttttctgccttgtttatagatcaataatcttcctaaaaggcacagtgagtgaatgaaataaatatattgtaattcttgtcctaagtagtagaaagttttctgcttgtttctgcaatgctttgaatgtcccaaagtttcatcagctttcctagtcttacacatttcaaagtactgaacacactgttgaatggctgtagttaccagagacttatatttcgtttcaagaagtcttaatactgtagttctgctataatgtgcatgcatccactttttgaaccacacagccttggtatcaactaatgcaaaaaagtagatcggatccaaaatcttttgtgagacaacatggctttgattatgtttaactgttaacaaggacaaagtactctccacaatttcttccatatacttctctggatgacgaatccagaaagatggagcttctttctgatattcatttagaagacgaacctttttaagtaagcgagtcatattaggattagttatatctacaccagctgaaagagtaggaatatgattttccctagaaagaaagtatgactccaaatacttagctaagcttgtataaatttccttggtcatatgtaatggagaaagcaaaaatgtctgtgcacagaattttaaaatccggtcactaaacacaggatcaggatctgaaagagacacggtcagtttttcgcagagagtagtccaattttcacagttgaggacatcagatggaggagctgaacataatgtttgcaaggcttcatatctcacctctttaggttgcccaggatccaactggtctaaaatcaattgtaattttccttgacaaaatttgtaactctgattcaatgatgaatcactatcagagcaattgtctgtgcggtaactatggcttttctccttttggatttttttctgcctttcttgatttcgtgtctcatcttcttcaaacttgttaatcatagactcgaccacagctatcataatgttcttcaggtaatgcatcatttctttgtactctttagattcttgagttcttttagtgacctgctgtacaactgtatcatagccgcattcttcaccctgattccgatcagatgtgcatttttccatttcttcttcaatcatagaacccaaagtgttgcctatatgctgcctgaggtatttcacaaattcatagttgtgaaaattttcatcagtttcctccagatgtaaaagaatctcttcggcacactccagggaaggggcacccgtgattttctccttcacgctctggaacaaccgcctcagcatcgcctgcagcatcgcctggtcctcgctggagaaatgggccatccttactttggggaagcaggggtccgcgaggtctcgcctctggtactcttagttgctagccttcagtaccagcagacctcaggctctcccgactaacaacaaaagagacatcaggaatgatctgatgggaggacccgacgacggaacgccacgatgcgcgtgacgtcagctcgctgatgtggcttccttggtgggagggagtgcaactggtgtcctgggggcgcccagagaatgttcgggtgagccactctccttcgccgccgcgttgtaggtgggagggaagagagtacgaagagaaagtgatcaataaaagaaagatagtaaaagtgaaactgaaagtagcctgacgagcctcagttgaagagtgaatggtattgaaaagttgcagtgttgttttcctctaacggctaacacctattgagctcctacgccctaccaaacactttccttaccaagcaccctgctaggagctatgaagaactccctcactaagtaacagagagaaaaataaattaacgattacaatacagtgcaattaaatgtcatgctagaaaaaaaagatatgccaagtcggtgctgtggagacccagaattagtttcaacccaatagaggagttgaggaaagaagcaaagagagtaaactggacatgcaaagaataggggcctcagagtgtaggatatactggcacttgaggtaatcgggttagaaagaggagatgaggaagctaaagaagtaaattggtcacatctggaagggtctaatcttttggcac

SEQ ID NO: 14407 - RNA, 4370 nt, Homo sapiens
  source 1..4370: mol_type = other RNA
gctgggattacaggcatgagccaccgcgcctggccaggactaactcttaaacatgaataagaactaaaagtaagctagatctgattctataataaccttacaaaacaacaaatttacaaaaatgaattcacaaattgagctcatacctacttaaatatatcgttatacttctcagtatttacaatatgtatattcacaaagtaaatgttgttacagacacagaaaaacatcaagcccccctgctgtgtttaaaaataaataaaacctaaatttaaaccgtgtgtctcatgatctatgtgctctgcagtctaatgttccgcatgtctctcagcagcactgttcggtagttttgttccaaaatttccatgtattcaaaataatcactcactcgaaacccatgcagtgcttcttcttttaggaaaacttgcagatcttgagtctgagtgtgctgtagaatgtcttgctgtaaatgtttgaatacagctatacagatatacacttgataatcaggaccaaggaaaacacaagtagcaatataatggcagatttctatccaatctaagtaattccaaaaacactgggttatccattgcaggcaaatctgtgatggtgcaaaaccagacatgtgaaaagctgaaaacacaagaggcaactcagccttcagtagcatttcaatataatgggtgctgcaaaaatatactggatggatgccagattctacagtgtcattaggaaggtaactagaaatatgtagccttggcaaccaaagaaaagcagaagtcagaagcctggagaattgatgaagaaattggaatgttttttctttgtctcccaacattatcatgaacagagaagatacaaaccagtcatggccagcataattcccttgcaggcagagaagagaagattttatggaagtttgctgctgtttcaggaatctctcacaatgctttaaaacccaggtaagatcattttctgcaccatcttttaagagactgaggaatttgccatacctgacagtcattttaatgccaagctgctgcacagatgaaagactttcattcttcacatttgcatcagtagctgtatactccactgaagggaagtagcattcagatgggctttcagtgagatgaagcacaaatttttcaagtaattctattaaggcctctccactgattatatcaggtttggctttcatcattttgcaaaattgtctttggcagttttctatccattcagtttgtttatcagatattttgaggcataataaaagcttgtcaagatcattgttcactgaacgctgcatagctccagagacacagaatatggtattcttgttctttggccccatctcttgttttataccagcatttcttgtaatgtctgacagatagcagtttggcaatggatatgatgaaaacattggccaaggatatggattatcactcttttcgagtaacctcggaggcaaaatccgttccaatggcccaccaacaagatttattctaacaagaacatgatttctctccactgataagccatcaattataaagtccctgtggctctcagaaatctccaagatattttcttcttgagcatttagtaacatttcagatacctgatactgagcctctaacaggagaagagtgtccagatcacagcatatcacacttaataaccttagaccaaagatatgtgattgttcatagttgaataaagaacgaatcttagcttcagaattcaaaattataagtctatcaataatatcaataacacatgttgggacttcacgaagagaatattctgttttattaggaagatcttgattccttacaagctcataaatagcaggataggataacaagttcaccagtgctaaaaaagacttttgacagcttcggtcaataggatccactggagtagttctgggatgggttaccctaacatcatctcttccatattccagattggaccataattcagttataagttcattaataaaccctgacttttttagtgcaatgccacctgctgctgttgatgccactcgtgtaaccaaaactccatagccaaattttttatgcctgctgacctgtaatttttttgcatatcgattgaatataaatgtcacacattcattgatagcacctgttctttgaagaagtagtaatcctttgggggtggcagcaaaatgtagtaaatcatctaacaaattatcttcccaagccataatgttttgggattcctggcttactgaagaaacagaatcagaaccctctactggagtaggaattctttctgatagcaaacttgtctttttccatgcctttgctatagattcatgcaaattataagtgattaacacctgcaaaccttcacatgtactatatatgtgacgacacacagaaataaaagctcctttaaccacaggcaacatttctgatccagaaaatatagaaatatcttcatcgagaagttttttcgaaaactgggcaattatatgagcacctgtaggactttcttcagaagagttcatatttgctccataaaggagtaaaataagcccttcttctacagatgcaattcttgccaaaataccagctatatgaattaaagctgtctcagagcaatttggagatgcctcatttcctttcattaaattgtgaataggctgaagaagtgtctctattacaatgttgttatataagcattccactgcacattctttttgatcactgagtatccacagaacttcagtcaccatacttgcaggagagtaattctctgaatgggcagctgatgtcatctttggacaacttggtgagtaatagataagttgggtaaaaagaacaagcagatctatgagggataccaaaccttttttattcttcagcttaataggaaatagttttctgccttgtttatagatcaataatcttcctaaaaggcacagtgagtgaatgaaataaatatattgtaattcttgtcctaagtagtagaaagttttctgcttgtttctgcaatgctttgaatgtcccaaagtttcatcagctttcctagtcttacacatttcaaagtactgaacacactgttgaatggctgtagttaccagagacttatatttcgtttcaagaagtcttaatactgtagttctgctataatgtgcatgcatccactttttgaaccacacagccttggtatcaactaatgcaaaaaagtagatcggatccaaaatcttttgtgagacaacatggctttgattatgtttaactgttaacaaggacaaagtactctccacaatttcttccatatacttctctggatgacgaatccagaaagatggagcttctttctgatattcatttagaagacgaacctttttaagtaagcgagtcatattaggattagttatatctacaccagctgaaagagtaggaatatgattttccctagaaagaaagtatgactccaaatacttagctaagcttgtataaatttccttggtcatatgtaatggagaaagcaaaaatgtctgtgcacagaattttaaaatccggtcactaaacacaggatcaggatctgaaagagacacggtcagtttttcgcagagagtagtccaattttcacagttgaggacatcagatggaggagctgaacataatgtttgcaaggcttcatatctcacctctttaggttgcccaggatccaactggtctaaaatcaattgtaattttccttgacaaaatttgtaactctgattcaatgatgaatcactatcagagcaattgtctgtgcggtaactatggcttttctccttttggatttttttctgcctttcttgatttcgtgtctcatcttcttcaaacttgttaatcatagactcgaccacagctatcataatgttcttcaggtaatgcatcatttctttgtactctttagattcttgagttcttttagtgacctgctgtacaactgtatcatagccgcattcttcaccctgattccgatcagatgtgcatttttccatttcttcttcaatcatagaacccaaagtgttgcctatatgctgcctgaggtatttcacaaattcatagttgtgaaaattttcatcagtttcctccagatgtaaaagaatctcttcggcacactccagggaaggggcacccgtgattttctccttcacgctctggaacaaccgcctcagcatcgcctgcagcatcgcctggtcctcgctggagaaatgggccatctttggggaagcaggggtccgcgaggtctcgcctctggtactcttagttgctagccttcagtaccagcagacctcaggctctcccgactaacaacaaaagagacatcaggaatgatct

SEQ ID NO: 14408 - RNA, 4244 nt, Homo sapiens
  source 1..4244: mol_type = other RNA
gctgggattacaggcatgagccaccgcgcctggccaggactaactcttaaacatgaataagaactaaaagtaagctagatctgattctataataaccttacaaaacaacaaatttacaaaaatgaattcacaaattgagctcatacctacttaaatatatcgttatacttctcagtatttacaatatgtatattcacaaagtaaatgttgttacagacacagaaaaacatcaagcccccctgctgtgtttaaaaataaataaaacctaaatttaaaccgtgtgtctcatgatctatgtgctctgcagtctaatgttccgcatgtctctcagcagcactgttcggtagttttgttccaaaatttccatgtattcaaaataatcactcactcgaaacccatgcagtgcttcttcttttaggaaaacttgcagatcttgagtctgagtgtgctgtagaatgtcttgctgtaaatgtttgaatacagctatacagatatacacttgataatcaggaccaaggaaaacacaagtagcaatataatggcagatttctatccaatctaagtaattccaaaaacactgggttatccattgcaggcaaatctgtgatggtgcaaaaccagacatgtgaaaagctgaaaacacaagaggcaactcagccttcagtagcatttcaatataatgggtgctgcaaaaatatactggatggatgccagattctacagtgtcattaggaaggtaactagaaatatgtagccttggcaaccaaagaaaagcagaagtcagaagcctggagaattgatgaagaaattggaatgttttttctttgtctcccaacattatcatgaacagagaagatacaaaccagtcatggccagcataattcccttgcaggcagagaagagaagattttatggaagtttgctgctgtttcaggaatctctcacaatgctttaaaacccaggtaagatcattttctgcaccatcttttaagagactgaggaatttgccatacctgacagtcattttaatgccaagctgctgcacagatgaaagactttcattcttcacatttgcatcagtagctgtatactccactgaagggaagtagcattcagatgggctttcagtgagatgaagcacaaatttttcaagtaattctattaaggcctctccactgattatatcaggtttggctttcatcattttgcaaaattgtctttggcagttttctatccattcagtttgtttatcagatattttgaggcataataaaagcttgtcaagatcattgttcactgaacgctgcatagctccagagacacagaatatggtattcttgttctttggccccatctcttgttttataccagcatttcttgtaatgtctgacagatagcagtttggcaatggatatgatgaaaacattggccaaggatatggattatcactcttttcgagtaacctcggaggcaaaatccgttccaatggcccaccaacaagatttattctaacaagaacatgatttctctccactgataagccatcaattataaagtccctgtggctctcagaaatctccaagatattttcttcttgagcatttagtaacatttcagatacctgatactgagcctctaacaggagaagagtgtccagatcacagcatatcacacttaataaccttagaccaaagatatgtgattgttcatagttgaataaagaacgaatcttagcttcagaattcaaaattataagtctatcaataatatcaataacacatgttgggacttcacgaagagaatattctgttttattaggaagatcttgattccttacaagctcataaatagcaggataggataacaagttcaccagtgctaaaaaagacttttgacagcttcggtcaataggatccactggagtagttctgggatgggttaccctaacatcatctcttccatattccagattggaccataattcagttataagttcattaataaaccctgacttttttagtgcaatgccacctgctgctgttgatgccactcgtgtaaccaaaactccatagccaaattttttatgcctgctgacctgtaatttttttgcatatcgattgaatataaatgtcacacattcattgatagcacctgttctttgaagaagtagtaatcctttgggggtggcagcaaaatgtagtaaatcatctaacaaattatcttcccaagccataatgttttgggattcctggcttactgaagaaacagaatcagaaccctctactggagtaggaattctttctgatagcaaacttgtctttttccatgcctttgctatagattcatgcaaattataagtgattaacacctgcaaaccttcacatgtactatatatgtgacgacacacagaaataaaagctcctttaaccacaggcaacatttctgatccagaaaatatagaaatatcttcatcgagaagttttttcgaaaactgggcaattatatgagcacctgtaggactttcttcagaagagttcatatttgctccataaaggagtaaaataagcccttcttctacagatgcaattcttgccaaaataccagctatatgaattaaagctgtctcagagcaatttggagatgcctcatttcctttcattaaattgtgaataggctgaagaagtgtctctattacaatgttgttatataagcattccactgcacattctttttgatcactgagtatccacagaacttcagtcaccatacttgcaggagagtaattctctgaatgggcagctgatgtcatctttggacaacttggtgagtaatagataagttgggtaaaaagaacaagcagatctatgagggataccaaaccttttttattcttcagcttaataggaaatagttttctgccttgtttatagatcaataatcttcctaaaaggcacagtgagtgaatgaaataaatatattgtaattcttgtcctaagtagtagaaagttttctgcttgtttctgcaatgctttgaatgtcccaaagtttcatcagctttcctagtcttacacatttcaaagtactgaacacactgttgaatggctgtagttaccagagacttatatttcgtttcaagaagtcttaatactgtagttctgctataatgtgcatgcatccactttttgaaccacacagccttggtatcaactaatgcaaaaaagtagatcggatccaaaatcttttgtgagacaacatggctttgattatgtttaactgttaacaaggacaaagtactctccacaatttcttccatatacttctctggatgacgaatccagaaagatggagcttctttctgatattcatttagaagacgaacctttttaagtaagcgagtcatattaggattagttatatctacaccagctgaaagagtaggaatatgattttccctagaaagaaagtatgactccaaatacttagctaagcttgtataaatttccttggtcatatgtaatggagaaagcaaaaatgtctgtgcacagaattttaaaatccggtcctctttaggttgcccaggatccaactggtctaaaatcaattgtaattttccttgacaaaatttgtaactctgattcaatgatgaatcactatcagagcaattgtctgtgcggtaactatggcttttctccttttggatttttttctgcctttcttgatttcgtgtctcatcttcttcaaacttgttaatcatagactcgaccacagctatcataatgttcttcaggtaatgcatcatttctttgtactctttagattcttgagttcttttagtgacctgctgtacaactgtatcatagccgcattcttcaccctgattccgatcagatgtgcatttttccatttcttcttcaatcatagaacccaaagtgttgcctatatgctgcctgaggtatttcacaaattcatagttgtgaaaattttcatcagtttcctccagatgtaaaagaatctcttcggcacactccagggaaggggcacccgtgattttctccttcacgctctggaacaaccgcctcagcatcgcctgcagcatcgcctggtcctcgctggagaaatgggccatctttggggaagcaggggtccgcgaggtctcgcctctggtactcttagttgctagccttcagtaccagcagacctcaggctctcccgactaacaacaaaagagacatcaggaatgatct

SEQ ID NO: 14409 - RNA, 3173 nt, Homo sapiens
  source 1..3173: mol_type = other RNA
gctgggattacaggcatgagccaccgcgcctggccaggactaactcttaaacatgaataagaactaaaagtaagctagatctgattctataataaccttacaaaacaacaaatttacaaaaatgaattcacaaattgagctcatacctacttaaatatatcgttatacttctcagtatttacaatatgtatattcacaaagtaaatgttgttacagacacagaaaaacatcaagcccccctgctgtgtttaaaaataaataaaacctaaatttaaaccgtgtgtctcatgatctatgtgctctgcagtctaatgttccgcatgtctctcagcagcactgttcggtagttttgttccaaaatttccatgtattcaaaataatcactcactcgaaacccatgcagtgcttcttcttttaggaaaacttgcagatcttgagtctgagtgtgctgtagaatgtcttgctgtaaatgtttgaatacagctatacagatatacacttgataatcaggaccaaggaaaacacaagtagcaatataatggcagatttctatccaatctaagtaattccaaaaacactgggttatccattgcaggcaaatctgtgatggtgcaaaaccagacatgtgaaaagctgaaaacacaagaggcaactcagccttcagtagcatttcaatataatgggtgctgcaaaaatatactggatggatgccagattctacagtgtcattaggaaggtaactagaaatatgtagccttggcaaccaaagaaaagcagaagtcagaagcctggagaattgatgaagaaattggaatgttttttctttgtctcccaacattatcatgaacagagaagatacaaaccagtcatggccagcataattcccttgcaggcagagaagagaagattttatggaagtttgctgctgtttcaggaatctctcacaatgctttaaaacccaggtaagatcattttctgcaccatcttttaagagactgaggaatttgccatacctgacagtcattttaatgccaagctgctgcacagatgaaagactttcattcttcacatttgcatcagtagctgtatactccactgaagggaagtagcattcagatgggctttcagtgagatgaagcacaaatttttcaagtaattctattaaggcctctccactgattatatcaggtttggctttcatcattttgcaaaattgtctttggcagttttctatccattcagtttgtttatcagatattttgaggcataataaaagcttgtcaagatcattgttcactgaacgctgcatagctccagagacacagaatatggtattcttgttctttggccccatctcttgttttataccagcatttcttgtaatgtctgacagatagcagtttggcaatggatatgatgaaaacattggccaaggatatggattatcactcttttcgagtaacctcggaggcaaaatccgttccaatggcccaccaacaagatttattctaacaagaacatgatttctctccactgataagccatcaattataaagtccctgtggctctcagaaatctccaagatattttcttcttgagcatttagtaacatttcagatacctgatactgagcctctaacaggagaagagtgtccagatcacagcatatcacacttaataaccttagaccaaagatatgtgattgttcatagttgaataaagaacgaatcttagcttcagaattcaaaattataagtctatcaataatatcaataacacatgttgggacttcacgaagagaatattctgttttattaggaagatcttgattccttacaagctcataaatagcaggataggataacaagttcaccagtgctaaaaaagacttttgacagcttcggtcaataggatccactggagtagttctgggatgggttaccctaacatcatctcttccatattccagattggaccataattcagttataagttcattaataaaccctgacttttttagtgcaatgccacctgctgctgttgatgccactcgtgtaaccaaaactccatagccaaattttttatgcctgctgacctgtaatttttttgcatatcgattgaatataaatgtcacacattcattgatagcacctgttctttgaagaagtagtaatcctttgggggtggcagcaaaatgtagtaaatcatctaacaaattatcttcccaagccataatgttttgggattcctggcttactgaagaaacagaatcagaaccctctactggagtaggaattctttctgatagcaaacttgtctttttccatgcctttgctatagattcatgcaaattataagtgattaacacctgcaaaccttcacatgtactatatatgtgacgacacacagaaataaaagctcctttaaccacaggcaacatttctgatccagaaaatatagaaatatcttcatcgagaagttttttcgaaaactgggcaattatatgagcacctgtaggactttcttcagaagagttcatatttgctccataaaggagtaaaataagcccttcttctacagatgcaattcttgccaaaataccagctatatgaattaaagctgtctcagagcaatttggagatgcctcatttcctttcattaaattgtgaataggctgaagaagtgtctctattacaatgttgttatataagcattccactgcacattctttttgatcactgagtatccacagaacttcagtcaccatacttgcaggagagtaattctctgaatgggcagctgatgtcatctttggacaacttggtgagtaatagataagttgggtaaaaagaacaagcagatctatgagggataccaaaccttttttattcttcagcttaataggaaatagttttctgccttgtttatagatcaataatcttcctaaaaggcacagtgagtgaatgaaataaatatattgtaattcttgtcctaagtagtagaaagttttctgcttgtttctgcaatgctttgaatgtcccaaagtttcatcagctttcctagtcttacacatttcaaagtactgaacacactgttgaatggctgtagttacctttctagcccttaaagctcagcctcctcaattacattttaactatggcatcactctggtg

SEQ ID NO: 14410 - RNA, 2593 nt, Homo sapiens
  source 1..2593: mol_type = other RNA
gctgggattacaggcatgagccaccgcgcctggccaggactaactcttaaacatgaataagaactaaaagtaagctagatctgattctataataaccttacaaaacaacaaatttacaaaaatgaattcacaaattgagctcatacctacttaaatatatcgttatacttctcagtatttacaatatgtatattcacaaagtaaatgttgttacagacacagaaaaacatcaagcccccctgctgtgtttaaaaataaataaaacctaaatttaaaccgtgtgtctcatgatctatgtgctctgcagtctaatgttccgcatgtctctcagcagcactgttcggtagttttgttccaaaatttccatgtattcaaaataatcactcactcgaaacccatgcagtgcttcttcttttaggaaaacttgcagatcttgagtctgagtgtgctgtagaatgtcttgctgtaaatgtttgaatacagctatacagatatacacttgataatcaggaccaaggaaaacacaagtagcaatataatggcagatttctatccaatctaagtaattccaaaaacactgggttatccattgcaggcaaatctgtgatggtgcaaaaccagacatgtgaaaagctgaaaacacaagaggcaactcagccttcagtagcatttcaatataatgggtgctgcaaaaatatactggatggatgccagattctacagtgtcattaggaaggtaactagaaatatgtagccttggcaaccaaagaaaagcagaagtcagaagcctggagaattgatgaagaaattggaatgttttttctttgtctcccaacattatcatgaacagagaagatacaaaccagtcatggccagcataattcccttgcaggcagagaagagaagattttatggaagtttgctgctgtttcaggaatctctcacaatgctttaaaacccaggtaagatcattttctgcaccatcttttaagagactgaggaatttgccatacctgacagtcattttaatgccaagctgctgcacagatgaaagactttcattcttcacatttgcatcagtagctgtatactccactgaagggaagtagcattcagatgggctttcagtgagatgaagcacaaatttttcaagtaattctattaaggcctctccactgattatatcaggtttggctttcatcattttgcaaaattgtctttggcagttttctatccattcagtttgtttatcagatattttgaggcataataaaagcttgtcaagatcattgttcactgaacgctgcatagctccagagacacagaatatggtattcttgttctttggccccatctcttgttttataccagcatttcttgtaatgtctgacagatagcagtttggcaatggatatgatgaaaacattggccaaggatatggattatcactcttttcgagtaacctcggaggcaaaatccgttccaatggcccaccaacaagatttattctaacaagaacatgatttctctccactgataagccatcaattataaagtccctgtggctctcagaaatctccaagatattttcttcttgagcatttagtaacatttcagatacctgatactgagcctctaacaggagaagagtgtccagatcacagcatatcacacttaataaccttagaccaaagatatgtgattgttcatagttgaataaagaacgaatcttagcttcagaattcaaaattataagtctatcaataatatcaataacacatgttgggacttcacgaagagaatattctgttttattaggaagatcttgattccttacaagctcataaatagcaggataggataacaagttcaccagtgctaaaaaagacttttgacagcttcggtcaataggatccactggagtagttctgggatgggttaccctaacatcatctcttccatattccagattggaccataattcagttataagttcattaataaaccctgacttttttagtgcaatgccacctgctgctgttgatgccactcgtgtaaccaaaactccatagccaaattttttatgcctgctgacctgtaatttttttgcatatcgattgaatataaatgtcacacattcattgatagcacctgttctttgaagaagtagtaatcctttgggggtggcagcaaaatgtagtaaatcatctaacaaattatcttcccaagccataatgttttgggattcctggcttactgaagaaacagaatcagaaccctctactggagtaggaattctttctgatagcaaacttgtctttttccatgcctttgctatagattcatgcaaattataagtgattaacacctgcaaaccttcacatgtactatatatgtgacgacacacagaaataaaagctcctttaaccacaggcaacatttctgatccagaaaatatagaaatatcttcatcgagaagttttttcgaaaactgggcaattatatgagcacctttcttcagaagagttcatatttgctccataaaggagtaaaataagcccttcttctacagatgcaattcttgccaaaatac

SEQ ID NO: 14411 - RNA, 4247 nt, Homo sapiens
  source 1..4247: mol_type = other RNA
gctgggattacaggcatgagccaccgcgcctggccaggactaactcttaaacatgaataagaactaaaagtaagctagatctgattctataataaccttacaaaacaacaaatttacaaaaatgaattcacaaattgagctcatacctacttaaatatatcgttatacttctcagtatttacaatatgtatattcacaaagtaaatgttgttacagacacagaaaaacatcaagcccccctgctgtgtttaaaaataaataaaacctaaatttaaaccgtgtgtctcatgatctatgtgctctgcagtctaatgttccgcatgtctctcagcagcactgttcggtagttttgttccaaaatttccatgtattcaaaataatcactcactcgaaacccatgcagtgcttcttcttttaggaaaacttgcagatcttgagtctgagtgtgctgtagaatgtcttgctgtaaatgtttgaatacagctatacagatatacacttgataatcaggaccaaggaaaacacaagtagcaatataatggcagatttctatccaatctaagtaattccaaaaacactgggttatccattgcaggcaaatctgtgatggtgcaaaaccagacatgtgaaaagctgaaaacacaagaggcaactcagccttcagtagcatttcaatataatgggtgctgcaaaaatatactggatggatgccagattctacagtgtcattaggaaggtaactagaaatatgtagccttggcaaccaaagaaaagcagaagtcagaagcctggagaattgatgaagaaattggaatgttttttctttgtctcccaacattatcatgaacagagaagatacaaaccagtcatggccagcataattcccttgcaggcagagaagagaagattttatggaagtttgctgctgtttcaggaatctctcacaatgctttaaaacccaggtaagatcattttctgcaccatcttttaagagactgaggaatttgccatacctgacagtcattttaatgccaagctgctgcacagatgaaagactttcattcttcacatttgcatcagtagctgtatactccactgaagggaagtagcattcagatgggctttcagtgagatgaagcacaaatttttcaagtaattctattaaggcctctccactgattatatcaggtttggctttcatcattttgcaaaattgtctttggcagttttctatccattcagtttgtttatcagatattttgaggcataataaaagcttgtcaagatcattgttcactgaacgctgcatagctccagagacacagaatatggtattcttgttctttggccccatctcttgttttataccagcatttcttgtaatgtctgacagatagcagtttggcaatggatatgatgaaaacattggccaaggatatggattatcactcttttcgagtaacctcggaggcaaaatccgttccaatggcccaccaacaagatttattctaacaagaacatgatttctctccactgataagccatcaattataaagtcccttagaccaaagatatgtgattgttcatagttgaataaagaacgaatcttagcttcagaattcaaaattataagtctatcaataatatcaataacacatgttgggacttcacgaagagaatattctgttttattaggaagatcttgattccttacaagctcataaatagcaggataggataacaagttcaccagtgctaaaaaagacttttgacagcttcggtcaataggatccactggagtagttctgggatgggttaccctaacatcatctcttccatattccagattggaccataattcagttataagttcattaataaaccctgacttttttagtgcaatgccacctgctgctgttgatgccactcgtgtaaccaaaactccatagccaaattttttatgcctgctgacctgtaatttttttgcatatcgattgaatataaatgtcacacattcattgatagcacctgttctttgaagaagtagtaatcctttgggggtggcagcaaaatgtagtaaatcatctaacaaattatcttcccaagccataatgttttgggattcctggcttactgaagaaacagaatcagaaccctctactggagtaggaattctttctgatagcaaacttgtctttttccatgcctttgctatagattcatgcaaattataagtgattaacacctgcaaaccttcacatgtactatatatgtgacgacacacagaaataaaagctcctttaaccacaggcaacatttctgatccagaaaatatagaaatatcttcatcgagaagttttttcgaaaactgggcaattatatgagcacctgtaggactttcttcagaagagttcatatttgctccataaaggagtaaaataagcccttcttctacagatgcaattcttgccaaaataccagctatatgaattaaagctgtctcagagcaatttggagatgcctcatttcctttcattaaattgtgaataggctgaagaagtgtctctattacaatgttgttatataagcattccactgcacattctttttgatcactgagtatccacagaacttcagtcaccatacttgcaggagagtaattctctgaatgggcagctgatgtcatctttggacaacttggtgagtaatagataagttgggtaaaaagaacaagcagatctatgagggataccaaaccttttttattcttcagcttaataggaaatagttttctgccttgtttatagatcaataatcttcctaaaaggcacagtgagtgaatgaaataaatatattgtaattcttgtcctaagtagtagaaagttttctgcttgtttctgcaatgctttgaatgtcccaaagtttcatcagctttcctagtcttacacatttcaaagtactgaacacactgttgaatggctgtagttaccagagacttatatttcgtttcaagaagtcttaatactgtagttctgctataatgtgcatgcatccactttttgaaccacacagccttggtatcaactaatgcaaaaaagtagatcggatccaaaatcttttgtgagacaacatggctttgattatgtttaactgttaacaaggacaaagtactctccacaatttcttccatatacttctctggatgacgaatccagaaagatggagcttctttctgatattcatttagaagacgaacctttttaagtaagcgagtcatattaggattagttatatctacaccagctgaaagagtaggaatatgattttccctagaaagaaagtatgactccaaatacttagctaagcttgtataaatttccttggtcatatgtaatggagaaagcaaaaatgtctgtgcacagaattttaaaatccggtcactaaacacaggatcaggatctgaaagagacacggtcagtttttcgcagagagtagtccaattttcacagttgaggacatcagatggaggagctgaacataatgtttgcaaggcttcatatctcacctctttaggttgcccaggatccaactggtctaaaatcaattgtaattttccttgacaaaatttgtaactctgattcaatgatgaatcactatcagagcaattgtctgtgcggtaactatggcttttctccttttggatttttttctgcctttcttgatttcgtgtctcatcttcttcaaacttgttaatcatagactcgaccacagctatcataatgttcttcaggtaatgcatcatttctttgtactctttagattcttgagttcttttagtgacctgctgtacaactgtatcatagccgcattcttcaccctgattccgatcagatgtgcatttttccatttcttcttcaatcatagaacccaaagtgttgcctatatgctgcctgaggtatttcacaaattcatagttgtgaaaattttcatcagtttcctccagatgtaaaagaatctcttcggcacactccagggaaggggcacccgtgattttctccttcacgctctggaacaaccgcctcagcatcgcctgcagcatcgcctggtcctcgctggagaaatgggccatctttggggaagcaggggtccgcgaggtctcgcctctggtactcttagttgctagccttcagtaccagcagacctcaggctctcccgactaacaacaaaagagacatcaggaatgatct

SEQ ID NO: 14412 - RNA, 4503 nt, Homo sapiens
  source 1..4503: mol_type = other RNA
gctgggattacaggcatgagccaccgcgcctggccaggactaactcttaaacatgaataagaactaaaagtaagctagatctgattctataataaccttacaaaacaacaaatttacaaaaatgaattcacaaattgagctcatacctacttaaatatatcgttatacttctcagtatttacaatatgtatattcacaaagtaaatgttgttacagacacagaaaaacatcaagcccccctgctgtgtttaaaaataaataaaacctaaatttaaaccgtgtgtctcatgatctatgtgctctgcagtctaatgttccgcatgtctctcagcagcactgttcggtagttttgttccaaaatttccatgtattcaaaataatcactcactcgaaacccatgcagtgcttcttcttttaggaaaacttgcagatcttgagtctgagtgtgctgtagaatgtcttgctgtaaatgtttgaatacagctatacagatatacacttgataatcaggaccaaggaaaacacaagtagcaatataatggcagatttctatccaatctaagtaattccaaaaacactgggttatccattgcaggcaaatctgtgatggtgcaaaaccagacatgtgaaaagctgaaaacacaagaggcaactcagccttcagtagcatttcaatataatgggtgctgcaaaaatatactggatggatgccagattctacagtgtcattaggaaggtaactctattttccttttgctgtaaattgctgcttcaaaattaatatggtggcataacaaatcacttccaagactcaggaaaaaagttaataatttataatcttggcaacttaaatccttgtggaaagatgaggagggagaaatatgtagccttggcaaccaaagaaaagcagaagtcagaagcctggagaattgatgaagaaattggaatgttttttctttgtctcccaacattatcatgaacagagaagatacaaaccagtcatggccagcataattcccttgcaggcagagaagagaagattttatggaagtttgctgctgtttcaggaatctctcacaatgctttaaaacccaggtaagatcattttctgcaccatcttttaagagactgaggaatttgccatacctgacagtcattttaatgccaagctgctgcacagatgaaagactttcattcttcacatttgcatcagtagctgtatactccactgaagggaagtagcattcagatgggctttcagtgagatgaagcacaaatttttcaagtaattctattaaggcctctccactgattatatcaggtttggctttcatcattttgcaaaattgtctttggcagttttctatccattcagtttgtttatcagatattttgaggcataataaaagcttgtcaagatcattgttcactgaacgctgcatagctccagagacacagaatatggtattcttgttctttggccccatctcttgttttataccagcatttcttgtaatgtctgacagatagcagtttggcaatggatatgatgaaaacattggccaaggatatggattatcactcttttcgagtaacctcggaggcaaaatccgttccaatggcccaccaacaagatttattctaacaagaacatgatttctctccactgataagccatcaattataaagtccctgtggctctcagaaatctccaagatattttcttcttgagcatttagtaacatttcagatacctgatactgagcctctaacaggagaagagtgtccagatcacagcatatcacacttaataaccttagaccaaagatatgtgattgttcatagttgaataaagaacgaatcttagcttcagaattcaaaattataagtctatcaataatatcaataacacatgttgggacttcacgaagagaatattctgttttattaggaagatcttgattccttacaagctcataaatagcaggataggataacaagttcaccagtgctaaaaaagacttttgacagcttcggtcaataggatccactggagtagttctgggatgggttaccctaacatcatctcttccatattccagattggaccataattcagttataagttcattaataaaccctgacttttttagtgcaatgccacctgctgctgttgatgccactcgtgtaaccaaaactccatagccaaattttttatgcctgctgacctgtaatttttttgcatatcgattgaatataaatgtcacacattcattgatagcacctgttctttgaagaagtagtaatcctttgggggtggcagcaaaatgtagtaaatcatctaacaaattatcttcccaagccataatgttttgggattcctggcttactgaagaaacagaatcagaaccctctactggagtaggaattctttctgatagcaaacttgtctttttccatgcctttgctatagattcatgcaaattataagtgattaacacctgcaaaccttcacatgtactatatatgtgacgacacacagaaataaaagctcctttaaccacaggcaacatttctgatccagaaaatatagaaatatcttcatcgagaagttttttcgaaaactgggcaattatatgagcacctgtaggactttcttcagaagagttcatatttgctccataaaggagtaaaataagcccttcttctacagatgcaattcttgccaaaataccagctatatgaattaaagctgtctcagagcaatttggagatgcctcatttcctttcattaaattgtgaataggctgaagaagtgtctctattacaatgttgttatataagcattccactgcacattctttttgatcactgagtatccacagaacttcagtcaccatacttgcaggagagtaattctctgaatgggcagctgatgtcatctttggacaacttggtgagtaatagataagttgggtaaaaagaacaagcagatctatgagggataccaaaccttttttattcttcagcttaataggaaatagttttctgccttgtttatagatcaataatcttcctaaaaggcacagtgagtgaatgaaataaatatattgtaattcttgtcctaagtagtagaaagttttctgcttgtttctgcaatgctttgaatgtcccaaagtttcatcagctttcctagtcttacacatttcaaagtactgaacacactgttgaatggctgtagttaccagagacttatatttcgtttcaagaagtcttaatactgtagttctgctataatgtgcatgcatccactttttgaaccacacagccttggtatcaactaatgcaaaaaagtagatcggatccaaaatcttttgtgagacaacatggctttgattatgtttaactgttaacaaggacaaagtactctccacaatttcttccatatacttctctggatgacgaatccagaaagatggagcttctttctgatattcatttagaagacgaacctttttaagtaagcgagtcatattaggattagttatatctacaccagctgaaagagtaggaatatgattttccctagaaagaaagtatgactccaaatacttagctaagcttgtataaatttccttggtcatatgtaatggagaaagcaaaaatgtctgtgcacagaattttaaaatccggtcactaaacacaggatcaggatctgaaagagacacggtcagtttttcgcagagagtagtccaattttcacagttgaggacatcagatggaggagctgaacataatgtttgcaaggcttcatatctcacctctttaggttgcccaggatccaactggtctaaaatcaattgtaattttccttgacaaaatttgtaactctgattcaatgatgaatcactatcagagcaattgtctgtgcggtaactatggcttttctccttttggatttttttctgcctttcttgatttcgtgtctcatcttcttcaaacttgttaatcatagactcgaccacagctatcataatgttcttcaggtaatgcatcatttctttgtactctttagattcttgagttcttttagtgacctgctgtacaactgtatcatagccgcattcttcaccctgattccgatcagatgtgcatttttccatttcttcttcaatcatagaacccaaagtgttgcctatatgctgcctgaggtatttcacaaattcatagttgtgaaaattttcatcagtttcctccagatgtaaaagaatctcttcggcacactccagggaaggggcacccgtgattttctccttcacgctctggaacaaccgcctcagcatcgcctgcagcatcgcctggtcctcgctggagaaatgggccatctttggggaagcaggggtccgcgaggtctcgcctctggtactcttagttgctagccttcagtaccagcagacctcaggctctcccgactaacaacaaaagagacatcaggaatgatct

SEQ ID NO: 14413 - RNA, 1629 nt, Homo sapiens
  source 1..1629: mol_type = other RNA
gctgggattacaggcatgagccaccgcgcctggccaggattttatttttttaagagggtcttgctatgctgcccaggctggcctcaaactcctgggctccagcaatcctcccacctcagcctctcaagtagttggaactacaggcatgagccacgatgcctggcttgttatcaggactgttgatctttacaattctcagggtaatgttttaaaaatcagctttatcaaggtataatttcatatgatacccaggtagttttgatttgcatttccccctttaagaaatgaggctccacctcgtttcataagcttaaatgatgagaagatttcacggtccctcaaggagaaatactgtcctgcttggtatcttacctttgcacaaattcccagtttgtgccaggcagtaacacaccctgtttatcttaaattcccaggtacagtcgtttgggtcttcactggttttaatcctaaggctgtatgagcttcatgtacattatcctgtctgttgcccataacacttctatgagatgatgatgatgatttccattctaagaatgaggaagcagaggagacacaagtaagccagaggcaatgctgggtttagaccctggttggcttgaggccacagcccataatcttctcactctctcactccaacttgaattggaatcagaccaccaagacgcccaccacagcttggccattagttgctgtgagacagtgagaaaatcccttcccctttctggtctctgtgcaatgagtggatggagttgctgacttccatgagctggatgggagaacagggcaggaaatgatccaggactgtgaagctgtcagtctcctccttgttcatcagagtgagtaagtagcaaagcaaaggaaaagcaaaactcccactccccaaaatgcaggcagcatccattcagtcctgaattccggggaaaggcgagagatggggacaggtccatatttcaagcgtttatccaacatatgcagggcaggccagcctcctcaagaggctttctttgtcccaggaacaaattacaaaggcaggtggaagtagttatcctcgttgaaagaaacaggcacaggaacttgctcagaggccctctctcaaaggtgccactccatattgaccacagttctggctgcattctgtcattggggtgggtggatgagctgtgctgggtcgagcctggtggtgcattgtgtgggtctcgagttcttgtcctgcagtcctaagttcttgtcctgcactgtagccagggtgtccggaggagtgttcggcccctagcagagagggtagctcctctctccagctggtagtccagtcatccctgtgtcctcagctctgctctgctccggctgagcccacggcttttatgggcctcagagggaaggaagtgagcaccaattggtccgtgggcagacacaggcgggccagaaaagacacaagtctccactctggtccataggattggcagcccagtccccagccttcagaccttccttggcctgaaagtggagcctcaccagggacctgcccccctccacccaggagcccatctgcctgctgtgctgaccaaggcacccaggctgcttgtaccaatgggcacctgcaggccagca

SEQ ID NO: 14414 - RNA, 4629 nt, Homo sapiens
  source 1..4629: mol_type = other RNA
gctgggattacaggcatgagccaccgcgcctggcccactagctctagtttttatcacacattgtcacctcagatattcataaaggttagatgttgcaaaataataaactctgtccacaataaacacaggcactttactaaaaatgctcatatagacctgtggttatcatctaaaaccatcttctagaaatggagatactagcaaagagcccttcccttcgcccttcctcttctccctctttcaccatccccagtgactaagtataggacgtctagctccaagaagtggactaataaaggtcactcccagaagacaggccttcctaaaaactaacaataggacattcacaaagggactgattcactacatctatttttaacatactttgagcattaagacttgtttatcctttaatacacaatattaacacaataaaatgcatacatagaacaatggttagaccatctgaactaatctaactcaggggcacagaacccttctccctgcatacctcctcctcctccccaccccaccacgcagtgaatagtcagcatacgctcctaagcatcaagttttaacaattccattcccaaatgcaaccactcctaggaagtactgaaaacaaatgcttagaggggtgttactttagccctctacttttaacctatgttgtggaatttttttttttttttttttttgagatggagtcttgctctgtcgccatgctggagtgcagtggtgtggtctcggcttactgcaacctctgtctcccgggctcaagcgattctcctgcctcagcctcccgagtagctgggactacaggcatgtgccaccacgaccagctaatttttgtattttttgtagagatggggtttcaccatgttggccaagatagtctcgatcccttgacttcgtgatctgcccacctcagcctcccaaagtgccaggattacaggagtgagccaccgcacctgaccattgtgcacttttaaacacctagaaagactagatgtttcaaactgcacttaagttttccattatatacacagtagtattgaataaatggcatatatacataacatagactataatttgagtgtcttctaaataggaacattctggcctagaacacttccctttctgacctctaccaaccccgttgacagctataagccatctgtaatgcttgggggcggggggcgtttaacaattttacttctgtttttaagaagtgttccttatgaattttaacacaaagtgtactcaatgtattagtttactaactctacttttgccatacactggcaacctctttaacatcgactagatataaattaggactcctatgtctgcttatatacacagcacagtaaacgaaaatgcagacataagggacaatggtcaatgtgcctcatcataaacacactggacactggtagaaagccctttgaactttgtgctccttcttccccctgaaccagcacaaatatcataacgtgtacttctcagagaattgatcaatttccaagacaatatttcatatcaaaataactacaaaatgtgttacttactacctctacttttaacatgctttgtgcacttctaaacatctagaaagactagatatttcaaataaggacttaagtgtgtccactatatacatagcactgttgaataaactacacacatgtaacaatggttatatctgaaagtgtcttctaaataggaacattctggtctagaacccttcattccttccaactcctctccaccaccaacctggtggatataagcacatgtgtcacttcgagctgatgttatcatttcacttccaaaaagtccttttcagaagacagcctctctatgaattttaacaaagtgtacaaaatgcgttagtttactaactacttttgtcatacactggcaacctctttaatagctacagactagatattataaaatcaggactcatttgtccagtatatacacaatatatacagtatagcaaagttaaatgaaatgcttgtaacatataggcaatggattaagctgaaattttctaataaacaatggcaaaacaccttttgcaattttttccctcccacctcccaggtggttcaacaaatccacttccaaacagcatttcccatcagtttttaaaagctatttacaaaaagtgttattctactactactactttaaaatacatcaagcacttccaaatatctaaagactagatatttcatagcctgtccaccatgtacacggcactgttaaataaaactgcacacacataacaatggttatcatctaaggtatcttctaaatgtgaccattttggccttgaatcattccctcttctcttccttctctgccttcaattcagtggacaagtacacgcatgtgtaatgcttagagatggctgaacaaattcctatgcaaaagtcaattacagaagacaagttttcctatgaatttcaacacaaagcatacaaaatatgctaattttactactttgtcatacactggcaacctctagatgttaaaaaattaagactatttgtccattatatacactatatacagagcaaaacaaaatgcacaaaacatacagaaaaatggtgtctgaaaatgtccaagtatgaacacactagcatattatcttttgcaatttcttccctcccacctcctctaaaccattgagcaagtatagacagtaatatactgctcacaaaggtggcttcacaattcaacttccaaaagtatttcctatgaattttagcaaaaagatatttacaaattggtattttactacctctacatttaatatacatcgggcacttctaaacatctagatagtctaaatgtttcaagtaaggagttaatttgtccactatgtatgtacacagcagtctcgaataaactgcaaacatgtaacaacagttataatttgaaagagtcttccaaatgtgaacattctggcctagaacccttcccatctccatcaacccagtgggcaagaatgctcaaattttcagaagacagtctttcctaggacttgtaaaacaaaatgtacaaaatatattagtttactaactctagttttgttatacactggcaacctctttaacatccagaaagactagatgttgtaaattaggactcgtttgtcctttatgtacattatatacatagataaaacaaaatgcacagacatagtgattcatcttgcctcgctgtaagcaggatggcatagagctctctgcacctccccctcctctctcctcccctgaactactgcacaaacacaatgagtattactcaacaggtgatttggccattccccccaaaaaacaacatttctatgaattgtaacaaaaagatatttacaaaatgtggttttactacctctaattttaacatatatcagacacttcagaatatctaaaaagaatagacatttcaaaaaagcttagcattgtcaactacatacatagtagtgaggaagcgaatgcacacaaaacaatggatagaatatgaaaatgtcttctaaatatgaccagtctagcatagaaccttctttttttccttctcaggtcttcgagctccatgtcatctaacccactgaacaaacgtgaacgtatcgcttctagaggccgtctaacaactcagtttccaaaagtcaactccggaagacatgtattttctatgatttcttttaaacaaatgagaatttacaagatgtgtgactttctaactctatcatacgtcggcaacctctttccatctagaagggctagatgtgacaaatgttttctattaaaaggttggggtggagttgagagcagctttttcatattatatacacaggccttccgtaaacggcctgtgaatcttcccagaggatggagggcatttccaacgggccaaacgtggcctgtcattctaccatttgtctcttccgacagcaaggtctggtagtacggagaccaaccgcccgatcgccgctaaccgttccacccgtcgtcgttcgggacttcgctcacctcccaggcccgttaaggcctttgtccgttgtcgttaggactaggtaggtctcgcccaatggcgacagagtggtcacccgggacccagatctggcggctccgtggcctgaagaggcggccgagcctgcctgcgtccctaggccgccttcccgggccctccatgccctaacgccctccgccgcgcggcgttcgagcggccgccatgcttcccggcacgctactcccgccgccacccaaaggcgctgcgtccaggctgctcggcgggggtttcgtccaggcccggcaggcttgggccgggagacccgacggccggcagggtccggactgggagaggccgccgccgccatcagtcaccgaggtagggtagggaagagacgttcgccaccgcttcaaggcctgggcccagccagtgggcagccacagcagaggcctccggtatctgcagggcagagggcgcggcctgtcccggggcgccccctagctcacccgccgacccggggccggagggcctggagcgccctggaggagcggcccgcgctctgcgtctctccgcgctctctgccagaccggaactcttgcagtg

SEQ ID NO: 14415 - RNA, 1994 nt, Homo sapiens
  source 1..1994: mol_type = other RNA
gctgggattacaggcatgagccaccgcgcctggccccaggttaatttttaacatgactgtgaactctcagagactcctgaagaataaacaaaagcctctctcgcctcattgtccccgagggagagagcccggtgccctgcgagggagaggctgagggtccagaggaaacgggaggctttccacggccactgcaagtgtttgctttaaacaaatatttcaaaagtcaagatcccgagagcagccatatgcctccttctgaggacccatgagtctctttcatctgcagtttattcagtgggactttggccttctccgacttctgaaggtcaaccagccgaagccaacacaccctctttacattgactcacagcgcaggccaagtccgcttgagtggaacatgcttctgagagtgaatttcctgccctggcagaatcaggtgctcctgcacagagtttgctcccagtgatggaggtgtcacatgctgtcctgagagttgagatggtcgatacagtgtttgaacttcacagagcacatcaggcccacaggagtaaaaggaagaactttattttccaaagcgtccccttgcctccctcctggagcttgaccctctgtaaatgagaaccattggctcttcccagtgtaaatcaaagtgtgtgcttacagatgtccctgtgaaaatgaaactatctgggccctgccttttataaacagaaaaaacaaaacaaagtgtctggtgaaggccattccttgggcttcattcagcacccacgaggctctgggaagagcccatccatgcgggagatattattaccaatggacccaaagaacaattggtggatgacagggtggacaacatgaaatagacaaaccagcactggaagagcgcccgggctgtgccccctgccccgcatcccccacccaccgccctacaaggtcagcctgtgcaacgtcggccccacgcaggcggcctctccaggtcgaggggtttccgtcggtgctcagagccatgcaactgcccttccagaggtggacaggctccaggggtgccggtcagccctgtgcaggcccgagagggctgtggaggcaggtttcaatgcgtgttttgtttggggctctttaaccttctcacagggaagccaggcccacaggggacagtgtaaaggaacacagcaaactttcactggcgctgggatggcatttgaggcctggtgacccacagacccgggctgcactctgcctccatggctggtctgtagggtggaaatgctcctgacaggcaagcttgatggactgtgagtatttcttccatgacgataatatttgaggtttaaagaaaaatcacaagtacatgtgttaggacgttaggagtgcttttggggcaggcgtattataattaagtggttatgtaaaacttttaaaaatgtgattagtttccactgtttctgttcttgttttcatctccagcagaaaagcaattcagagtcagtctcagggagcggagagaaggctgggaatctcagctttgctgaaggtaattgcggggccctgaggaaatcatttaatttcttgacatgccgtttgtgcacaggactgacccaatggcttccttgtatggccgtcctgggtagcaaaggcatccgcacgcatgagctgtggtgggtatggtgatgcctggtgaggcacatgctccatgcaccatggatgctatcttctttaggtatgtcctgaaagacttgacttctcggccgggcgcggtggctcacacctgtaatcccagcttgggaggccaaggcaggcggatcacaaggtcaggagatcaagaccatcctggataacacggtaaaaccccgtctctacatgtgagagccctgagggtgggacagccgtggcctcctgcttgccggtcacagagccacacacacactccaaggcagggttcctggaagccgaggcctgcacaggaacccagggggatgctggggttgaagaggaac

SEQ ID NO: 14416 - RNA, 3932 nt, Homo sapiens
  source 1..3932: mol_type = other RNA
gctgggattacaggcatgagccaccgcgcctggcctacattcactctttagcgagatgatttgttgtcaatataagcaagtagtgctgtgaaaatgaggcagcattataatcctagttatgctgtaaccagatttacaaccagaattcaggattaacccatttgtatgatcattaatcctattctttcagaaatagacacattgtttctggttgtatttcagaagaaaaacagagaagccattctatctttaggcaggggtgactgcaggacttgagtgtgcacaaattttggtaaatgcaggggtcctgaaaccaatccctggagtataccaagggatgatgtcgttttcaatcaagcaagacattctcaattggggacctgggtataacttttctctagaaatgaagtacaacttcattcactccagtgtgaaatatatgggaaaagtccccaagatcaaagcctgtgttgtatataatatctagaaaattgttggcacttaggaaaaaaataaataaaaagaaaagatataaaaacttttggtcaaaaaaacctgtatttttcagtatgtacattccaaatgaatgtttttatattgagttcatttagaatgctttgtctttaaaaattcactttaaacacagactactataggtagttcaatttttagatttttttttaagtggtcagagttcagttaaagattacttactttacacactgctaaaatttttgagaaaaaatataaactcattttaatcaccatggttatgtaagcacatcaaaaaaattttcactcagaatagcactgtttttatgtcagattttacacagatcatacctatacatgcctccatgcaatgatcatttctatagactaagataattaaaactgcatttttaaacaaaataatctgtcatatatttttttgatctcagttgtgatcatgattattatcatatcaaaaaagatttttataaaccatgaaaatctctttattatttcatttgtctgcatcaatatttcaaaatatattggcctggttctgtagcttttaggtaaaccatttccaggatcaaagagatcctcaattccggctatatgtaataacacttcattattagatactaagcaaatttgcatttttaaaactccaatttattatccaaagtattttcaaaggcttttattgataaatgcattaatcattttatttcagcatttactaaatgtgaccttacatggtgatcagtgcagctcatggatatccaggtcagtcaaaaactgatttttctttatgattaatcattcgtgactcgcttgaccacagaggctgttgggtcagcactcactctaactgaacagagatatgccagggcccacgtgaacattattagcaaatctgtgatgtagatcagcagcgtattataacaccagcttaccctggacgctgccaaatcgtctgaataattctagccattttgcccatgttagggataaggtgtttattttataaataaagcctagaagcagtcttagtgcttctctttcaatggcttaatagaaaaaagaatgagtgttttgagtctgaagaaatagtcaatgcattgaggaagttttgtcttgtattccttgctcatagagacctcccgaacccactttcaggatgcaagtgtacgcatagcctcatcctggacatcaagttcttcttccgtcagctctgtttctattaattcaagggtatctttacaatcctgaatgagagtgatcgtttctaaaatggaaccttgaccctcttgagatttcacttggttctgtagatagagtatagcatcatggaccgtcaaaaagaatgtgtcctttctaatgttgtcgtcaaagaacccgcattgctccagcttttctatcacataatcttgaagtgatgcaaaatacacattcacatcaattctttggaattctttgacaatcacccgcagtgatctcactccaacaacgtccaggaaagatatagctccacagtcaagcacaaggctatggattggcactttgggaacgttcactttgactggaagctcagagttccaatccacttgaatctctatttccttggttgggatatcaagttcctccagatcttcaatatcctcatcaggctcaaaagcattatttgttgaaacagcatcacttatgatgccattctttgttgctcttaattgtccactttttattagtttctgtattttcctcagcgctttcagcctcttattatatactctaatggcatcaaatccaactgtggacttgatacattttttaaaaccatcgacattgccatagaaaataggactggaaaatctaagaatcttcactccttgaggttcttcaatgtttttgtaattcttggtacttttgtagatatctgtgctagggatgcttccaaggccattccaagaaggaaactgaactctcaggaccacagtcaacagtccaaatataaggccagctagtaaaccgagatccagccccagaatgatggacactatacacgtaaacacccagataacagcatcaatcttattctgtctccacagacgaggaatgtcacacagctgcataaacatccctttcaggttggcaattacaacagctgccaagaccgactgtgtctttcctccagtgctctcctggacggccgtgcgggaaagagcagtggtggccacaaaacaagagaagaatcctgagaagatgttgctgatcccaaaggcaatgaattcctggttcccatcgatggtgtaatcatacttggtggcatatacttttcctactgacactgcaatagcataagccaccacagcgatggaaaatgatgcagccagcatctccgagaacaagctcacaggtggaagttcaggaggcaaaaacccccttgggatggatttaacaatgccagcattgtaatttttttccaggttggctccatatgaaatggcagtagcaattatcgtcacaattacttctataggaatagggactgggattttgtgtctaaaccgatcatttaattccttaactgccatacagacgacaatggtgagcaatccagcagtgaaatcagcaagattggtatcaccaatattttgaaaaatctcaaccagcgtatagataatagagagaactccattgtagtttttggttgaaacattgaggacaatctttagctgtgagaccagcacttggaaggcagcagctgttgtgaagccaccaaccaaaggatctgccaagtacctcactatgaatccaatctgcaagccaccaaatatcaactgtataattccaaccagcagagtcagggcactggcaatcaggactctagctgtatctctagctgcagtgtctatcatagtagtatttaatacagttccattgctgctggatacgagaaagtgttcgtcgggggccatgctcagaacaacagatcccaccattaaactcaccactggaaaaggtccaactgagatatgtcttgatgttccaaagataaagtatgtcaggatagggaaaaaagcagagtagagaccatatccgacaggaactgcagctagtagggcatatgccatcccttgcagcgtggccactagcccagtactaactcccgaaatgacgtcactaagcagccattccttgactcggtatttggggagccactccaagatgggcacaagagtctttagcacaccaaaggctctctttcttgaacaactgcagcacttggccaggctctcccgcagcgtcttgcgctcctgcaggcgccgctcgtgctgttgctggaaagcgagctcgctgtagaccggccgcgacaccatgtagctgcagctgtactcggggagctgcggcggctccgacctgccgcctggcgctgccatgac

SEQ ID NO: 14417 - RNA, 4214 nt, Homo sapiens
  source 1..4214: mol_type = other RNA
gctgggattacaggcatgagccaccgcgcctggcctacattcactctttagcgagatgatttgttgtcaatataagcaagtagtgctgtgaaaatgaggcagcattataatcctagttatgctgtaaccagatttacaaccagaattcaggattaacccatttgtatgatcattaatcctattctttcagaaatagacacattgtttctggttgtatttcagaagaaaaacagagaagccattctatctttaggcaggggtgactgcaggacttgagtgtgcacaaattttggtaaatgcaggggtcctgaaaccaatccctggagtataccaagggatgatgtcgttttcaatcaagcaagacattctcaattggggacctgggtataacttttctctagaaatgaagtacaacttcattcactccagtgtgaaatatatgggaaaagtccccaagatcaaagcctgtgttgtatataatatctagaaaattgttggcacttaggaaaaaaataaataaaaagaaaagatataaaaacttttggtcaaaaaaacctgtatttttcagtatgtacattccaaatgaatgtttttatattgagttcatttagaatgctttgtctttaaaaattcactttaaacacagactactataggtagttcaatttttagatttttttttaagtggtcagagttcagttaaagattacttactttacacactgctaaaatttttgagaaaaaatataaactcattttaatcaccatggttatgtaagcacatcaaaaaaattttcactcagaatagcactgtttttatgtcagattttacacagatcatacctatacatgcctccatgcaatgatcatttctatagactaagataattaaaactgcatttttaaacaaaataatctgtcatatatttttttgatctcagttgtgatcatgattattatcatatcaaaaaagatttttataaaccatgaaaatctctttattatttcatttgtctgcatcaatatttcaaaatatattggcctggttctgtagcttttaggtaaaccatttccaggatcaaagagatcctcaattccggctatatgtaataacacttcattattagatactaagcaaatttgcatttttaaaactccaatttattatccaaagtattttcaaaggcttttattgataaatgcattaatcattttatttcagcatttactaaatgtgaccttacatggtgatcagtgcagctcatggatatccaggtcagtcaaaaactgatttttctttatgattaatcattcgtgactcgcttgaccacagaggctgttgggtcagcactcactctaactgaacagagatatgccagggcccacgtgaacattattagcaaatctgtgatgtagatcagcagcgtattataacaccagcttaccctggacgctgccaaatcgtctgaataattctagccattttgcccatgttagggataaggtgtttattttataaataaagcctagaagcagtcttagtgcttctctttcaatggcttaatagaaaaaagaatgagtgttttgagtctgaagaaatagtcaatgcattgaggaagttttgtcttgtattccttgctcatagagacctcccgaacccactttcaggatgcaagtgtacgcatagcctcatcctggacatcaagttcttcttccgtcagctctgtttctattaattcaagggtatctttacaatcctgaatgagagtgatcgtttctaaaatggaaccttgaccctcttgagatttcacttggttctgtagatagagtatagcatcatggaccgtcaaaaagaatgtgtcctttctaatgttgtcgtcaaagaacccgcattgctccagcttttctatcacataatcttgaagtgatgcaaaatacacattcacatcaattctttggaattctttgacaatcacccgcagtgatctcactccaacaacgtccaggaaagatatagctccacagtcaagcacaaggctatggattggcactttgggaacgttcactttgactggaagctcagagttccaatccacttgaatctctatttccttggttgggatatcaagttcctccagatcttcaatatcctcatcaggctcaaaagcattatttgttgaaacagcatcacttatgatgccattctttgttgctcttaattgtccactttttattagtttctgtattttcctcagcgctttcagcctcttattatatactctaatggcatcaaatccaactgtggacttgatacattttttaaaaccatcgacattgccatagaaaataggactggaaaatctaagaatcttcactccttgaggttcttcaatgtttttgtaattcttggtacttttgtagatatctgtgctagggatgcttccaaggccattccaagaaggaaactgaactctcaggaccacagtcaacagtccaaatataaggccagctagtaaaccgagatccagccccagaatgatggacactatacacgtaaacacccagataacagcatcaatcttattctgtctccacagacgaggaatgtcacacagctgcataaacatccctttcaggttggcaattacaacagctgccaagaccgacttctgcaagggttccagaagcttccccagggcaagaatggcgatcatcacaatcgcagcagagatgatgccagcaacctgtgtctttcctccagtgctctcctggacggccgtgcgggaaagagcagtggtggccacaaaacaagagaagaatcctgagaagatgttgctgatcccaaaggcaatgaattcctggttcccatcgatggtgtaatcatacttggtggcatatacttttcctactgacactgcaatagcataagccaccacagcgatggaaaatgatgcagccagcatctccgagaacaagctcacaggtggaagttcaggaggcaaaaacccccttgggatggatttaacaatgccagcattgtaatttttttccaggttggctccatatgaaatggcagtagcaattatcgtcacaattacttctataggaatagggactgggattttgtgtctaaaccgatcatttaattccttaactgccatacagacgacaatggtgagcaatccagcagtgaaatcagcaagattggtatcaccaatattttgaaaaatctcaaccagcgtatagataatagagagaactccattgtagtttttggttgaaacattgaggacaatctttagctgtgagaccagcacttggaaggcagcagctgttgtgaagccaccaaccaaaggatctgccaagtacctcactatgaatccaatctgcaagccaccaaatatcaactgtataattccaaccagcagagtcagggcactggcaatcaggactctagctgtatctctagctgcagtgtctatcatagtagtatttaatacagttccattgctgctggatacgagaaagtgttcgtcgggggccatgctcagaacaacagatcccaccattaaactcaccactggaaaaggtccaactgagatatgtcttgatgttccaaagataaagtatgtcaggatagggaaaaaagcagagtagagaccatatccgacaggaactgcagctagtagggcatatgccatcccttgcagcgtggccactagcccagtactaactcccgaaatgacgtcactaagcagccattccttgactcggtatttggggagccactccaagatgggcacaagagtctttagcacaccaaaggctctctttcttgaacaactgcagcacttggccaggctctcccgcagcgtcttgcgctcctgcaggcgccgctcgtgctgttgctggaaagcgagctcgctgtagaccggccgcgacaccatgtagctgcagctgtactcggggagctgcggcggctccgacctgccgcctggcgctgccatgacctgacccgggacgcagctccaggtgcgcactggaggagaggtgcagacccccgggccaggcgtggaaccgtcagggcgcgctccgcgggtccccaagaggcggacgctgcaggcacattccagcagctgtcgcagccctctcgggggcagaactttcagcttattgagcaagtctctcccctcgtcctgttttccgagcagcct

SEQ ID NO: 14418 - RNA, 4038 nt, Homo sapiens
  source 1..4038: mol_type = other RNA
gctgggattacaggcatgagccaccgcgcctggcctacattcactctttagcgagatgatttgttgtcaatataagcaagtagtgctgtgaaaatgaggcagcattataatcctagttatgctgtaaccagatttacaaccagaattcaggattaacccatttgtatgatcattaatcctattctttcagaaatagacacattgtttctggttgtatttcagaagaaaaacagagaagccattctatctttaggcaggggtgactgcaggacttgagtgtgcacaaattttggtaaatgcaggggtcctgaaaccaatccctggagtataccaagggatgatgtcgttttcaatcaagcaagacattctcaattggggacctgggtataacttttctctagaaatgaagtacaacttcattcactccagtgtgaaatatatgggaaaagtccccaagatcaaagcctgtgttgtatataatatctagaaaattgttggcacttaggaaaaaaataaataaaaagaaaagatataaaaacttttggtcaaaaaaacctgtatttttcagtatgtacattccaaatgaatgtttttatattgagttcatttagaatgctttgtctttaaaaattcactttaaacacagactactataggtagttcaatttttagatttttttttaagtggtcagagttcagttaaagattacttactttacacactgctaaaatttttgagaaaaaatataaactcattttaatcaccatggttatgtaagcacatcaaaaaaattttcactcagaatagcactgtttttatgtcagattttacacagatcatacctatacatgcctccatgcaatgatcatttctatagactaagataattaaaactgcatttttaaacaaaataatctgtcatatatttttttgatctcagttgtgatcatgattattatcatatcaaaaaagatttttataaaccatgaaaatctctttattatttcatttgtctgcatcaatatttcaaaatatattggcctggttctgtagcttttaggtaaaccatttccaggatcaaagagatcctcaattccggctatatgtaataacacttcattattagatactaagcaaatttgcatttttaaaactccaatttattatccaaagtattttcaaaggcttttattgataaatgcattaatcattttatttcagcatttactaaatgtgaccttacatggtgatcagtgcagctcatggatatccaggtcagtcaaaaactgatttttctttatgattaatcattcgtgactcgcttgaccacagaggctgttgggtcagcactcactctaactgaacagagatatgccagggcccacgtgaacattattagcaaatctgtgatgtagatcagcagcgtattataacaccagcttaccctggacgctgccaaatcgtctgaataattctagccattttgcccatgttagggataaggtgtttattttataaataaagcctagaagcagtcttagtgcttctctttcaatggcttaatagaaaaaagaatgagtgttttgagtctgaagaaatagtcaatgcattgaggaagttttgtcttgtattccttgctcatagagacctcccgaacccactttcaggatgcaagtgtacgcatagcctcatcctggacatcaagttcttcttccgtcagctctgtttctattaattcaagggtatctttacaatcctgaatgagagtgatcgtttctaaaatggaaccttgaccctcttgagatttcacttggttctgtagatagagtatagcatcatggaccgtcaaaaagaatgtgtcctttctaatgttgtcgtcaaagaacccgcattgctccagcttttctatcacataatcttgaagtgatgcaaaatacacattcacatcaattctttggaattctttgacaatcacccgcagtgatctcactccaacaacgtccaggaaagatatagctccacagtcaagcacaaggctatggattggcactttgggaacgttcactttgactggaagctcagagttccaatccacttgaatctctatttccttggttgggatatcaagttcctccagatcttcaatatcctcatcaggctcaaaagcattatttgttgaaacagcatcacttatgatgccattctttgttgctcttaattgtccactttttattagtttctgtattttcctcagcgctttcagcctcttattatatactctaatggcatcaaatccaactgtggacttgatacattttttaaaaccatcgacattgccatagaaaataggactggaaaatctaagaatcttcactccttgaggttcttcaatgtttttgtaattcttggtacttttgtagatatctgtgctagggatgcttccaaggccattccaagaaggaaactgaactctcaggaccacagtcaacagtccaaatataaggccagctagtaaaccgagatccagccccagaatgatggacactatacacgtaaacacccagataacagcatcaatcttattctgtctccacagacgaggaatgtcacacagctgcataaacatccctttcaggttggcaattacaacagctgccaagaccgacttctgcaagggttccagaagcttccccagggcaagaatggcgatcatcacaatcgcagcagagatgatgccagcaacctgtgtctttcctccagtgctctcctggacggccgtgcgggaaagagcagtggtggccacaaaacaagagaagaatcctgagaagatgttgctgatcccaaaggcaatgaattcctggttcccatcgatggtgtaatcatacttggtggcatatacttttcctactgacactgcaatagcataagccaccacagcgatggaaaatgatgcagccagcatctccgagaacaagctcacaggtggaagttcaggaggcaaaaacccccttgggatggatttaacaatgccagcattgtaatttttttccaggttggctccatatgaaatggcagtagcaattatcgtcacaattacttctataggaatagggactgggattttgtgtctaaaccgatcatttaattccttaactgccatacagacgacaatggtgagcaatccagcagtgaaatcagcaagattggtatcaccaatattttgaaaaatctcaaccagcgtatagataatagagagaactccattgtagtttttggttgaaacattgaggacaatctttagctgtgagaccagcacttggaaggcagcagctgttgtgaagccaccaaccaaaggatctgccaagtacctcactatgaatccaatctgcaagccaccaaatatcaactgtataattccaaccagcagagtcagggcactggcaatcaggactctagctgtatctctagctgcagtgtctatcatagtagtatttaatacagttccattgctgctggatacgagaaagtgttcgtcgggggccatgctcagaacaacagatcccaccattaaactcaccactggaaaaggtccaactgagatatgtcttgatgttccaaagataaagtatgtcaggatagggaaaaaagcagagtagagaccatatccgacaggaactgcagctagtagggcatatgccatcccttgcagcgtggccactagcccagtactaactcccgaaatgacgtcactaagcagccattccttgactcggtatttggggagccactccaagatgggcacaagagtctttagcacaccaaaggctctctttcttgaacaactgcagcacttggccaggctctcccgcagcgtcttgcgctcctgcaggcgccgctcgtgctgttgctggaaagcgagctcgctgtagaccggccgcgacaccatgtagctgcagctgtactcggggagctgcggcggctccgacctgccgcctggcgctgccatgacctgtctctgctcgcgccccgcccggaat

SEQ ID NO: 14419 - RNA, 549 nt, Homo sapiens
  source 1..549: mol_type = other RNA
gctgggattacaggcatgagccaccgcgcctggcctccaaaagaattttccaaaatggtgattctcccattaagacaaacggtcatgggaacgtaggcaagccactctgaattctctccaagaccttccactgtggcctgttgcgcatctgcagaatcctgcagcagattgggaatcaggggccatttcaaacacgtgttattaagtcaggagcccagtatgcactaagtgtcgtgggagcacagccagccagtgtgaccccacgctgggggcaaggagccttgcaccaggactacacagcctgagttccttcttgacttgaccactttgtcttggacctgtggtttgccttttcttactgtcagtgtcttcaccttgctgacaccttgatcttggacttcccagcctccagaactgtgagaaataaatttttgttgtttaatccatccagtctgtgatattttgttatggcagctgaagcagtcaggaaaggatcctccccatctctgcagaagcctgaccatccccctagagggcctgggaggaagt

SEQ ID NO: 14420 - RNA, 2777 nt, Homo sapiens
  source 1..2777: mol_type = other RNA
gctgggattacaggcatgagccaccgcgcctggcctcctgccacctttctgatctgtttgttttgtgtgtgtgcattgcctgtctcccccaactagaggataaactattttgtggctgggcctcattgtcttattcattgctccatctcatggtttagcccaaagcctggcattcagtggatgcccaataaatacttggtgaataaatgaatgaatgacaattaccctagccagactgaacgactggtccttctgcccagagcactccccacttgctcccccaccccacccttttgtatagcttagtcaccggtcagatctcattttcggcatcacttcctgcaggaagtcctccctgatctcctctctctagagtgggctggttgtcctccagcatcattctgtgttgcccttactgttgcacttctcagaagctatggcaattgtgtgctttctttctggcctcccccacctggctgtgagctccttgaggacagggttacatttatcctctgtgtgtcccctctgcctagaagagacgctaccaggatgagagggtatataccttacagttacaagcaagaatatgggcaccagacttgcctgagttctaatctcaatggtaccagtctatggaactttgagtccattcttcaacctctctgtgcctcagctctctaatctataaaatggtcacaaatacagtgcccatgttgtttctctgacacagagtaaatggtcaattacatgttaaatgttagcagctagtatttgtaggaacctagtaaaatagtcattgaataaattaatgaccagatacggtggctcacacctataatccaagcacttagggaagctgaagcgggaggatagcttgaggccaggagttcaagaccagcctgggcagcacagtgagacctcttctctactaaaagaagtcaagctgggcgtagtggtgcacctatagtctcagctactcgggaggctgaggcaggaggatcacttgagcccaggagtttgaggctgcagtgagctgtgattgttccactgcactccagcctgggtgatagagtgagactctgtctctaaaataaatacagaaaaacccagtgatttttatctgggagctttgagactgacttccttaaataggttgctttagggtttctcacagtgctgtgcatgccttagactcacagacaccttcacacccacaccagtaactccacctcctgctcagggaacacgattgccctgaggggtgaacctcctccccccaccttttttttttttttttgctatccctagagggcagcatgagcctggtatgcagtagatgctcaataaataacatgtcttgttttcattcgttcaaacatgatactctatttttgagtacctccctcccttttgagaagccagatccccttatttcccatctcagatccccaggtcccacctgggctgccttatgggatggagtctcctggagccaacttccctgagcctcccagccccaactggcatggccctcgagtctccccacgtggtatcccctgcctttgcagtgacctacacactcgcctctgagccaagatggcagcaagaaacccgttgcccctccccgtcatgctggggcattctgaccactgctctggcctgccctggggtaagatgacagcaggtggccctggggagggtggattttctcagggctggccccttctcatcttttagatcacactttgttgcctgcgcagagaggcccttaccaagcactgcatcaggaaaggtcttcaccccaatcactctccctctagcatcctgtttcagttcctgcagagcattcatcgctgttcaaaatcatcttctttatttattgggttactttatttattcagggtgggttccctccaccccaaaaataccagctccaggaaaaccatggtatctccccagcactttgcagggcctggcatgtggaagatgtaccagtaatatttgctgtatgaatgaatgagtctcttcatgtgcaggtgacttatcctgcctctgccactcgacggatgtttcagatgccccttagcggatctaatgatgtttccttggctcaagcacaaaagactcctgcttagctggggaagcagggccaggccctgggaattgcagcctctgggcatcagagcccggcccttccagctaatcggcctgcccacagacacaagaggagagggctttcagtgagtccttgactgttccccaagttgaagacctcacaggcgcagccttcacgggtttccccttagcctcgggaacctcctgggggcagagcgggctgactgggaaggaagctgaggccacagaccctctgcagagcggcagggtggccctggcctgggcaaggcatcccccacccatgggggtcacccgagtcagatggggccagttttccccacagaacacgatgtaggtcttcattggtggggtgacaagccctcgattgggactgggggcttggggtggtgatgcggttgctgccagggagagctgcttcccgtgggtgcagtcaataacaaaagtcaggtgagccgtggggacggtcttctgatggccagccagcttcccaccggagctggtctccaggcctgtctcacggatggtgcctttgaggttggctctccagtccctggggtcttctgacggggccatgcggctacttcggcgcctgcctagctctggcaggagaggagctgtcctaggccactcttccaggatgt

SEQ ID NO: 14421 - RNA, 629 nt, Homo sapiens
  source 1..629: mol_type = other RNA
gctgggattacaggcatgagccaccgcgcctggcctgaggtttgctttttgtgtaagatggtgcctttccttctggttgtttaggtggcagctttgactccagatctacaaaggcagagattcacagtccacagataattagaaagtcagcctgttcactagggtgcaggaagagcttcctcattcctttgttggctctttctctcctgcagtcatcgggttagggtgaacccttcctctcagcatcatgcttcaatcatcatcatcatcatcatcatcatcatggtcatcatcatcataggctttccttactcaccaatccacatgaagcaaagggagccacccccactagatcacttgagagtatccttacctgcacataactctttgttggctcaggttacatgagacttaggatcttcagtgatgctcacccccaagttggggtgattcctcagccttatgctacctacagaatatgaatggtgatgataatagtaatatctaagatttgtaagtagttgtgtgtcagatcccattctaagcacgtttacatatattaactcatttaattcttgctgctttatgacatagatactattattatccccattttataaatgaagaaa

SEQ ID NO: 14422 - RNA, 404 nt, Homo sapiens
  source 1..404: mol_type = other RNA
gctgggattacaggcatgagccaccgcgcctggcctgtgccgctcctcaggcggctctccgtgagctccgagatggctccggcagtggcggtcttcttcaggcgaaccacccccgatgcagcggtacttcctggcttgttgagcgtgtcctcactgctggccctcttgagcctgctgagtcgggactcaaaagccaaggaagttgaagacttagaactcttcatgccggaagaggctgcaggcagaggccgcacccggtctgggccgtggccccctgctctgatggctgggttccagggcttggctgcactccgcatgcttgacttcgtgggtctgtccggccccgctggctcagcgccgccgcaacccccagcggccacggctccgggcgctcactgatgctc

SEQ ID NO: 14423 - RNA, 520 nt, Homo sapiens
  source 1..520: mol_type = other RNA
gctgggattacaggcatgagccaccgcgcctggcctgtgccgctcctcaggcggctctccgtgagctccgagatggctccggcagtggcggtcttcttcaggcgaaccacccccgatgcagcggtacttcctggcttgttgagcgtgtcctcactgctggccctcttgagcctgctgagtcgggactcaaaagccaaggaagttgaagacttagaactcttcatgccggaagaggctgcaggcagaggccgcacccggtctgggccgtggccccctgctctgatggctgggttccagggcttggctgcactccgcatgcttgacttcgtgggtctgtcctggggaactgcagtctgaatgaccaggactgttggacccttcccctcacatggaatacacacgccactcagcagcacaccacagctcttcaacaatcacaggaggcacgctacgccggccccgctggctcagcgccgccgcaacccccagcggccacggctccgggcgctcactgatgctc

SEQ ID NO: 14424 - RNA, 849 nt, Homo sapiens
  source 1..849: mol_type = other RNA
gctgggattacaggcatgagccaccgcgcctggctgacttcctcttttattacttatcttcttgaccctgccttggctgttgggctctaagagcatacaaattctaccacctccagctaccaatgcgagccaagttctgagccttgagtgggaatgtggcacaactgggcactgggtaattaagtcctgggtccaggccaaaggaggacccagccttatatggagttcataggacagaggcacatgactttcttaggaggcagccaaaggcctctggactgatcagggcatcggtggcagaggagcagggtgacaggccgcctttggctgggctttatctgggctgatgctgaagctgtagaggccctggagcacaccattcaccaccacgttgggcagcgactctggggaggggttgcaaacatagggatccacatggaagctcaggacaggccgctggtgctgctgggagctgctgtcgccaggcaggaactccctcagggtgccccagttgctagccttggggtctgtggggaagtgccgaagtctcaggaattccagtaactccttgggcacctcctggttcaggtacaggatgccctggatgtaagcctccaagccctgccggcgctgttccaaccctctggtcctccagttgggcaggcgtttcgaggggaagtcgggcactttgtacagcttcttgatcatgtggcttttctccgggctctgcctgggcccctcggcctcgggccccaccgacgggatgtgaacttccagcatccgcgccccggccccagctgctccgcgcgctcggctcggagccctaactctcccggagcggactgagga

SEQ ID NO: 14425 - RNA, 909 nt, Homo sapiens
  source 1..909: mol_type = other RNA
gctgggattacaggcatgagccaccgcgcctggctgacttcctcttttattacttatcttcttgaccctgccttggctgttgggctctaagagcatacaaattctaccacctccagctaccaatgcgagccaagttctgagccttgagtgggaatgtggcacaactgggcactgggtaattaagtcctgggtccaggccaaaggaggacccagccttatatggagttcataggacagaggcacatgactttcttaggaggcagccaaaggcctctggactgatcagggcatcggtggcagaggagcagggtgacaggccgcctttggctgggctttatctgggctgatgctgaagctgtagaggccctggagcacaccattcaccaccacgttgggcagcgactctggggaggggttgcaaacatagggatccacatggaagctcaggacaggccgctggtgctgctgggagctgctgtcgccaggcaggaactccctcagggtgccccagttgctagccttggggtctgtggggaagtgccgaagtctcaggaattccagtaactccttgggcacctcctggttcaggtacaggatgccctggatgtaagcctccaagccctgccggcgctgttccaaccctctggtcctccagttgggcaggcgtttcgaggggaagtcgggcactttgtacagcttcttgatccgcttgtgcagcgcgtggaactcgctgtagcgccttggcaccgtgtgtctgcgcccgctgcacagcacctccactcggaacaccatgtggcttttctccgggctctgcctgggcccctcggcctcgggccccaccgacgggatgtgaacttccagcatccgcgccccggccccagctgctccgcgcgctcggctcggagccct

SEQ ID NO: 14426 - RNA, 956 nt, Homo sapiens
  source 1..956: mol_type = other RNA
gctgggattacaggcatgagccaccgcgcctggctgacttcctcttttattacttatcttcttgaccctgccttggctgttgggctctaagagcatacaaattctaccacctccagctaccaatgcgagccaagttctgagccttgagtgggaatgtggcacaactgggcactgggtaattaagtcctgggtccaggccaaaggaggacccagccttatatggagttcataggacagaggcacatgactttcttaggaggcagccaaaggcctctggactgatcagggcatcggtggcagaggagcagggtgacaggccgcctttggctgggctttatctgggctgatgctgaagctgtagaggccctggagcacaccattcaccaccacgttgggcagcgactctggggaggggttgcaaacatagggatccacatggaagctcaggacaggccgctggtgctgctgggagctgctgtcgccaggcaggaactccctcagggtgctgctcactgctgacagcccctggcccccgccatcggccccccttacccccagttgctagccttggggtctgtggggaagtgccgaagtctcaggaattccagtaactccttgggcacctcctggttcaggtacaggatgccctggatgtaagcctccaagccctgccggcgctgttccaaccctctggtcctccagttgggcaggcgtttcgaggggaagtcgggcactttgtacagcttcttgatccgcttgtgcagcgcgtggaactcgctgtagcgccttggcaccgtgtgtctgcgcccgctgcacagcacctccactcggaacaccatgtggcttttctccgggctctgcctgggcccctcggcctcgggccccaccgacgggatgtgaacttccagcatccgcgccccggccccagctgctccgcgcgctcggctcggagccct

SEQ ID NO: 14427 - RNA, 4084 nt, Homo sapiens
  source 1..4084: mol_type = other RNA
gctgggattacaggcatgagccaccgcgcctggctgtttttaaccctagatgtaaattagaatcacttgggaaacttaaaaaatgtatgcctgggccctcctccagcaatttaaatcagaatctctgtaggcatcaaagctgagaaccacagaaataactatccttttcctgagctaagtccttcttgaaactaatctaatattgacaaacttctatttaagaaataccgactacaaccaacaaatgtttaatatgcagcaaatgaaaaaatcatgtctaggatactcaacccaagacatgagcacatcatgtacaaattcattgtaaacttacaaaataagtttcaaaatttctgcaagccctcactatacaaactcagaatcctctttatttttgagacagggtctggctctgtcacccagactggagtacagtggcacaatctcagcccactgcaacctccatctcctgggctcaggcgatcctctcacctcagcctcccaagtagctgggactatggtatgccaccaagcccggctgattttcatattttttgtagagatggggttttgccatgttggccaggctgctcttcaactcctgacctcaagggatccacccaccctggtctcccaaagtgctgggattacaggcatgagccactgtgccaggcctgttcttagggaaagctttttaggtttattaatgaaaatcctaatgttactaattgagacatcagttaacacccaacttagtgattcccatccaaccataattatgtatttttcaagaaaatacataatttactaacacattttccttaccatagccattttcaaaagaaggtagggtactaacactttccagtttagatggccaaagcccggtcagtctctataattaaacaattattttaaaccctagttatgctaaaaccaagctattcttatcacaagtcccattctgctaaccacaaaatttagagaatttgtacctggaagataccaccacgtgtcaattacaatatacgtattccttggtcaattctgatatcacaggaccggaaaaaatagctgcttggtgtctagattgtttgggtattaaaaccactgcacatggataagctatttgttcagtcggagagaaagggcatagagtgacagagcaacaaaaagacacacagagaatgtatttcttgtgaaagaaaagaatgaaatgaaatgaaatgtagaaaccctaatggccttttgctttggaaaattaactccacaagccactaaaaatactatcaattagatcagaaaagacattcggtatgtatgtgttcctcaagcattttagaaaggggatatgctataacttccctgttggttccagattcaacacagcacaaagcaagaaaacttttatttactacactcacaagtatgattaagtgttcctgtttactctggtaggttaaaatatcaaatattagttcccacagaagaacttttttttaaacatctaatcctattcgaaggataaaaggggaaaaactcattaaatgttgaacactgccactttaagtaccatttttgtcttcgggtgaatgtacataagactaaatcatgatccaacaatagttttctatttggtttcactagtatcactcaaagaacttgacacaggctaatgctttaacactttcttatctgagacaaatttaactctaagaacatatgactcaacaatgtacaaagatttaagaatttgccaatctgtcaatcattttaaagagtccatataatatacacatagcaatataatattcataaccagaaactgcactaagtaaacacatcatttagtttaagctctacctgaaaacatgctgttttattaaaacaaaacccaaagacttaaatctcaagttatatggttttacaattaagtcttactgaagcagcacagatttcctttcttacaaacaagttaatatgcaggaagaacccacaaagtgcacaccaacaatgtgacaaattgtaatatgtgaaatacaaataaatcctgaagttaatctgaagaatgtcaaggagttaccagagaggttatgtagtgcccttgatttttattttacctacaagtctacaaattctaaaatttactcaattgatttaacttttttaataaacagcaccagtcttgcccattgatacaattaaaatttgaccttctcagttcttagttcacaagtttattatgaaaaacactgcagtgctcttgtgcagtcacatcgtcttacaggaaggggaaaaaacagttctgttcaaaacaactcaccaggttctgacaataacaaagaacaacatggggctgagatttgagtagggaataaactgagtgcagacaaatcatataattaaattaaacggtatccctgaaaataaaaagaacaatttcaaaactcacaagtagaagggaggccttggtaattatttttaaaaatgttcattaagctccaatgattgtttgctgctatccttatctacagtcatgctgagtaaagctatagctaaatggaagttaaattgtattcacgaggtgttaatgtttacatcttattatctgcagtctctcagagaaagcaaaagtaactacaaatagcgctatgccagaaactggtttcttgaccaacaatgtcgcttcagcatgcaatgaactggttcattctaaagtggtcacggctgttgatgacaagaggctttgtatttttatatggcacatcttttggtccatgtgaaaacaagttttttgaatgttaactattttctgacactttggagttactgttgctcttcccatttccattaggtcgatatatggttcatggcaatactgtacaagtttaaaatttcattacaggaagtagtctggggtacgacgagtaacatgtggctcgcctctacgaggtgctgggtcaaactgcaagaaagagtattttagagtatcgtcaagttccatgattgcagcttggttaccacaacgataacaatagtttggagcactgaaaatcgttactacattccggtcatggcaccagttatatccctccatcactagctggtgagctctagacaccaacgtgaggccattggcatgattaaatgtctcagaaatatcttgcccaaaggtgtaaccagctcctcgaggagatataccccaaccaccacggtcatctggatctgaccacagcaagtcacacattggaccctaaaaaataactcatggggaacttcttgtaggcgatcaagtgctctgatatgatccagtgtatctatagatggcgagagaccaccatgtagacagaagatctgcccatccaccaaggcagtgagaggaagatagtcaaaaagatctgtaaaatatttccaaacatttgcatttccatattttcttaaacattcatcatagaaaccataaacttgtgtgatctgtctgctctcatgattccctcgaagaatggtgatgcgttcacggtaacgaaccttaagagctacaagcagtgtaactgtttcaactgaataatatcctctgtcaacataatctcccataaacaagtaatttgtatctggtgatttgccaccaattctaaacagttccatgagatcatgaaattgcccatgcacatctccacagacagtaactggacatcgaacctcttgcacgttggattcttttgtcaggatttctttagccttgatttctggagaagatcgcttggtgagtttaatacaaaccaccaaggggtactaaagctgtgtgacctttaggtatgttctgggatacggcctaacaagactgcctttgggggatcctctgggcagctctggacctaactaggcctgggtaccagcggcaagactcttactcagcccaccggagaggcccaggctccattcccaagccgcagaatccaagccagctcaccctcaaaaccgtccctgacgatgacccacagggtctccgctccccctgccacctcgtctggcgccaaggccggctgactcaaaagcccaggagtcgagtgaacggcgccatttt

SEQ ID NO: 14428 - RNA, 4041 nt, Homo sapiens
  source 1..4041: mol_type = other RNA
gctgggattacaggcatgagccaccgcgcctggctgtttttaaccctagatgtaaattagaatcacttgggaaacttaaaaaatgtatgcctgggccctcctccagcaatttaaatcagaatctctgtaggcatcaaagctgagaaccacagaaataactatccttttcctgagctaagtccttcttgaaactaatctaatattgacaaacttctatttaagaaataccgactacaaccaacaaatgtttaatatgcagcaaatgaaaaaatcatgtctaggatactcaacccaagacatgagcacatcatgtacaaattcattgtaaacttacaaaataagtttcaaaatttctgcaagccctcactatacaaactcagaatcctctttatttttgagacagggtctggctctgtcacccagactggagtacagtggcacaatctcagcccactgcaacctccatctcctgggctcaggcgatcctctcacctcagcctcccaagtagctgggactatggtatgccaccaagcccggctgattttcatattttttgtagagatggggttttgccatgttggccaggctgctcttcaactcctgacctcaagggatccacccaccctggtctcccaaagtgctgggattacaggcatgagccactgtgccaggcctgttcttagggaaagctttttaggtttattaatgaaaatcctaatgttactaattgagacatcagttaacacccaacttagtgattcccatccaaccataattatgtatttttcaagaaaatacataatttactaacacattttccttaccatagccattttcaaaagaaggtagggtactaacactttccagtttagatggccaaagcccggtcagtctctataattaaacaattattttaaaccctagttatgctaaaaccaagctattcttatcacaagtcccattctgctaaccacaaaatttagagaatttgtacctggaagataccaccacgtgtcaattacaatatacgtattccttggtcaattctgatatcacaggaccggaaaaaatagctgcttggtgtctagattgtttgggtattaaaaccactgcacatggataagctatttgttcagtcggagagaaagggcatagagtgacagagcaacaaaaagacacacagagaatgtatttcttgtgaaagaaaagaatgaaatgaaatgaaatgtagaaaccctaatggccttttgctttggaaaattaactccacaagccactaaaaatactatcaattagatcagaaaagacattcggtatgtatgtgttcctcaagcattttagaaaggggatatgctataacttccctgttggttccagattcaacacagcacaaagcaagaaaacttttatttactacactcacaagtatgattaagtgttcctgtttactctggtaggttaaaatatcaaatattagttcccacagaagaacttttttttaaacatctaatcctattcgaaggataaaaggggaaaaactcattaaatgttgaacactgccactttaagtaccatttttgtcttcgggtgaatgtacataagactaaatcatgatccaacaatagttttctatttggtttcactagtatcactcaaagaacttgacacaggctaatgctttaacactttcttatctgagacaaatttaactctaagaacatatgactcaacaatgtacaaagatttaagaatttgccaatctgtcaatcattttaaagagtccatataatatacacatagcaatataatattcataaccagaaactgcactaagtaaacacatcatttagtttaagctctacctgaaaacatgctgttttattaaaacaaaacccaaagacttaaatctcaagttatatggttttacaattaagtcttactgaagcagcacagatttcctttcttacaaacaagttaatatgcaggaagaacccacaaagtgcacaccaacaatgtgacaaattgtaatatgtgaaatacaaataaatcctgaagttaatctgaagaatgtcaaggagttaccagagaggttatgtagtgcccttgatttttattttacctacaagtctacaaattctaaaatttactcaattgatttaacttttttaataaacagcaccagtcttgcccattgatacaattaaaatttgaccttctcagttcttagttcacaagtttattatgaaaaacactgcagtgctcttgtgcagtcacatcgtcttacaggaaggggaaaaaacagttctgttcaaaacaactcaccaggttctgacaataacaaagaacaacatggggctgagatttgagtagggaataaactgagtgcagacaaatcatataattaaattaaacggtatccctgaaaataaaaagaacaatttcaaaactcacaagtagaagggaggccttggtaattatttttaaaaatgttcattaagctccaatgattgtttgctgctatccttatctacagtcatgctgagtaaagctatagctaaatggaagttaaattgtattcacgaggtgttaatgtttacatcttattatctgcagtctctcagagaaagcaaaagtaactacaaatagcgctatgccagaaactggtttcttgaccaacaatgtcgcttcagcatgcaatgaactggttcattctaaagtggtcacggctgttgatgacaagaggctttgtatttttatatggcacatcttttggtccatgtgaaaacaagttttttgaatgttaactattttctgacactttggagttactgttgctcttcccatttccattaggtcgatatatggttcatggcaatactgtacaagtttaaaatttcattacaggaagtagtctggggtacgacgagtaacatgtggctcgcctctacgaggtgctgggtcaaactgcaagaaagagtattttagagtatcgtcaagttccatgattgcagcttggttaccacaacgataacaatagtttggagcactgaaaatcgttactacattccggtcatggcaccagttatatccctccatcactagctggtgagctctagacaccaacgtgaggccattggcatgattaaatgtctcagaaatatcttgcccaaaggtgtaaccagctcctcgaggagatataccccaaccaccacggtcatctggatctgaccacagcaagtcacacattggaccctcatggggaacttcttgtaggcgatcaagtgctctgatatgatccagtgtatctatagatggcgagagaccaccatgtagacagaagatctgcccatccaccaaggcagtgagaggaagatagtcaaaaagatctgtaaaatatttccaaacatttgcatttccatattttcttaaacattcatcatagaaaccataaacttgtgtgatctgtctgctctcatgattccctcgaagaatggtgatgcgttcacggtaacgaaccttaagagctacaagcagtgtaactgtttcaactgaataatatcctctgtcaacataatctcccataaacaagtaatttgtatctggtgatttgccaccaattctaaacagttccatgagatcatgaaattgcccatgcacatctccacagacagtaactggacatcgaacctcttgcacgttggattcttttgtcaggatttctttagccttctcgcagaggctcttgacctgggactcggacagctgcttgcactcgttcagctgctcgatccactggtccagctccttggtgaacaccttctcgtccatgatgccacccgccccagccggctgccgctccgcgctgctcccgcgccgccgcccgcacacgggcctacacgcacacgccgccgccggttcctcgtgtacttctggcggctgttgaggctggcgctggcccgctggctctcaccgcagtactcggccgtcggccgctgcgcctcctcctccgctcgctgaggctccagagctcggctctctgt

SEQ ID NO: 14429 - RNA, 4073 nt, Homo sapiens
  source 1..4073: mol_type = other RNA
gctgggattacaggcatgagccaccgcgcctggctgtttttaaccctagatgtaaattagaatcacttgggaaacttaaaaaatgtatgcctgggccctcctccagcaatttaaatcagaatctctgtaggcatcaaagctgagaaccacagaaataactatccttttcctgagctaagtccttcttgaaactaatctaatattgacaaacttctatttaagaaataccgactacaaccaacaaatgtttaatatgcagcaaatgaaaaaatcatgtctaggatactcaacccaagacatgagcacatcatgtacaaattcattgtaaacttacaaaataagtttcaaaatttctgcaagccctcactatacaaactcagaatcctctttatttttgagacagggtctggctctgtcacccagactggagtacagtggcacaatctcagcccactgcaacctccatctcctgggctcaggcgatcctctcacctcagcctcccaagtagctgggactatggtatgccaccaagcccggctgattttcatattttttgtagagatggggttttgccatgttggccaggctgctcttcaactcctgacctcaagggatccacccaccctggtctcccaaagtgctgggattacaggcatgagccactgtgccaggcctgttcttagggaaagctttttaggtttattaatgaaaatcctaatgttactaattgagacatcagttaacacccaacttagtgattcccatccaaccataattatgtatttttcaagaaaatacataatttactaacacattttccttaccatagccattttcaaaagaaggtagggtactaacactttccagtttagatggccaaagcccggtcagtctctataattaaacaattattttaaaccctagttatgctaaaaccaagctattcttatcacaagtcccattctgctaaccacaaaatttagagaatttgtacctggaagataccaccacgtgtcaattacaatatacgtattccttggtcaattctgatatcacaggaccggaaaaaatagctgcttggtgtctagattgtttgggtattaaaaccactgcacatggataagctatttgttcagtcggagagaaagggcatagagtgacagagcaacaaaaagacacacagagaatgtatttcttgtgaaagaaaagaatgaaatgaaatgaaatgtagaaaccctaatggccttttgctttggaaaattaactccacaagccactaaaaatactatcaattagatcagaaaagacattcggtatgtatgtgttcctcaagcattttagaaaggggatatgctataacttccctgttggttccagattcaacacagcacaaagcaagaaaacttttatttactacactcacaagtatgattaagtgttcctgtttactctggtaggttaaaatatcaaatattagttcccacagaagaacttttttttaaacatctaatcctattcgaaggataaaaggggaaaaactcattaaatgttgaacactgccactttaagtaccatttttgtcttcgggtgaatgtacataagactaaatcatgatccaacaatagttttctatttggtttcactagtatcactcaaagaacttgacacaggctaatgctttaacactttcttatctgagacaaatttaactctaagaacatatgactcaacaatgtacaaagatttaagaatttgccaatctgtcaatcattttaaagagtccatataatatacacatagcaatataatattcataaccagaaactgcactaagtaaacacatcatttagtttaagctctacctgaaaacatgctgttttattaaaacaaaacccaaagacttaaatctcaagttatatggttttacaattaagtcttactgaagcagcacagatttcctttcttacaaacaagttaatatgcaggaagaacccacaaagtgcacaccaacaatgtgacaaattgtaatatgtgaaatacaaataaatcctgaagttaatctgaagaatgtcaaggagttaccagagaggttatgtagtgcccttgatttttattttacctacaagtctacaaattctaaaatttactcaattgatttaacttttttaataaacagcaccagtcttgcccattgatacaattaaaatttgaccttctcagttcttagttcacaagtttattatgaaaaacactgcagtgctcttgtgcagtcacatcgtcttacaggaaggggaaaaaacagttctgttcaaaacaactcaccaggttctgacaataacaaagaacaacatggggctgagatttgagtagggaataaactgagtgcagacaaatcatataattaaattaaacggtatccctgaaaataaaaagaacaatttcaaaactcacaagtagaagggaggccttggtaattatttttaaaaatgttcattaagctccaatgattgtttgctgctatccttatctacagtcatgctgagtaaagctatagctaaatggaagttaaattgtattcacgaggtgttaatgtttacatcttattatctgcagtctctcagagaaagcaaaagtaactacaaatagcgctatgccagaaactggtttcttgaccaacaatgtcgcttcagcatgcaatgaactggttcattctaaagtggtcacggctgttgatgacaagaggctttgtatttttatatggcacatcttttggtccatgtgaaaacaagttttttgaatgttaactattttctgacactttggagttactgttgctcttcccatttccattaggtcgatatatggttcatggcaatactgtacaagtttaaaatttcattacaggaagtagtctggggtacgacgagtaacatgtggctcgcctctacgaggtgctgggtcaaactgcaagaaagagtattttagagtatcgtcaagttccatgattgcagcttggttaccacaacgataacaatagtttggagcactgaaaatcgttactacattccggtcatggcaccagttatatccctccatcactagctggtgagctctagacaccaacgtgaggccattggcatgattaaatgtctcagaaatatcttgcccaaaggtgtaaccagctcctcgaggagatataccccaaccaccacggtcatctggatctgaccacagcaagtcacacattggaccctcatggggaacttcttgtaggcgatcaagtgctctgatatgatccagtgtatctatagatggcgagagaccaccatgtagacagaagatctgcccatccaccaaggcagtgagaggaagatagtcaaaaagatctgtaaaatatttccaaacatttgcatttccatattttcttaaacattcatcatagaaaccataaacttgtgtgatctgtctgctctcatgattccctcgaagaatggtgatgcgttcacggtaacgaaccttaagagctacaagcagtgtaactgtttcaactgaataatatcctctgtcaacataatctcccataaacaagtaatttgtatctggtgatttgccaccaattctaaacagttccatgagatcatgaaattgcccatgcacatctccacagacagtaactggacatcgaacctcttgcacgttggattcttttgtcaggatttctttagccttgatttctggagaagatcgcttggtgagtttaatacaaaccaccaaggggtactaaagctgtgtgacctttaggtatgttctgggatacggcctaacaagactgcctttgggggatcctctgggcagctctggacctaactaggcctgggtaccagcggcaagactcttactcagcccaccggagaggcccaggctccattcccaagccgcagaatccaagccagctcaccctcaaaaccgtccctgacgatgacccacagggtctccgctccccctgccacctcgtctggcgccaaggccggctgactcaaaagcccaggagtcgagtgaacggcgccatttt

SEQ ID NO: 14430 - RNA, 13930 nt, Homo sapiens
  source 1..13930: mol_type = other RNA
gctgggattacaggcatgagccaccgcgcgcgcccggccaactgagtagttgtagttctttatatagcctatactagtccttgtcagatccatgatttgcaaatatttttctcccattctgtgggtttttactttcttgctggtgtcctttgaagcaaaacgttttaattttgaagtgtagtttttttcttttgttgcctgtctttttatatcatatctaagacatcattgtgtaatccaaggtcatgaggatttaaaaaaaaatttatgggtacataattagcatatttatgaggtatatgagatgttttcatataggcatacgatgtaatcatcacaggagggtagatggggtttccatcacctcaagcattcatcatttctgtcatgaacattccaattgtacttcctcagttatttttgaaggtacaacaaattattgctgactgcagtcaccctgttgtgctatcaaatactagatatttttcaatcatggggattttcacctatattttctactaagagttttgtagtttcaactcttacatttaagtctttgactcattctgagctaatttttgtatatggtgtgagaaaggcatatcactttattcctttgcatgtggatatccagttgtcctaacaccatttgttaaaaagactattctttccctcatcaaattgtcttggcctccttgtcgaaaatcagttcactatagatgcaagggtttatttttgactctcagttctattctcttgatctgtatgtctatctacatttatctgtatatctgtctacaaactacacagatttgattaatacagctttgtaataaattttgaaatcaggaagtgcacatcctccaactttgttcttctttctccagatttatttgatcctttgtatttcaatatggattttagcgtcagcttagcttgtcaatttctttctcttttttttttttttttgttttttgtttttttgagacagagttttgctcttgttgctgaggatggagtgcagtggcatgatcttggctcactgcaacctctacctcctgcctcagcctcccaaatagctgagattacaggcatgcaccaccatgcctggctaattttgtatttttaatagagacagggttttaccatgttggccaagctggtcttgaattcctgacctcaagtaatccatctgccttggccgcccaaagtgctgggattacaggtgtgagccaccacacccggcccagcttgtcaatttctgcaaagaaggctgagattcttgatcaggattgtgttcaattggtagatcaatttggggcctattttcatcctaacaataattatctcccaatccataaacatgggatgtctttccatttatttaggtgttctttaatttctttcagagatgttttgtagtatttggtgtagaaatgaacttttgttaaatttattcctaagtatttcattctttttggtgttgatataaatggaattgttttcttaacttcaaattgtttgtaatatgtagaaataccattgagttttgtatattgatcttgtgtctggcaatcttgctaaactctttattagttctaacagcgtaagtggatttcttaggactttttctatatggtatcttgtcgtctgcaaagagagatcatcatacttctccctttccaatctgaatgcgcagtcttctttccttccttttgtcgaattgctctgtctagaacatttaatacaatgttgaagtgacaagaataaatatacttgttttgtgcctgatattgggaagaaagctcccaactggagctttcacatcaccattaatatgatgtaggctgtgggtttttccaaagatgctctttatcatgttgaggaagtaatttatttctagtttgttgaaaggttttttccaagaaagagtgttgtgtattgccaaatgctttttcagtgtatattgaaatgatcatgtgctttttgtcctcttttttctattaaagtggtatattatattaagtaaattttgtatgttaaaaaaaccttgcattctttcttttccccttctcaacgtttattttagaatcaggggggtacatgtgcgaatttgttacaaaggtatattgggtgatgctgaggtctggggtatggttgaacctgtcacccaggtagcgagcacagtatccaataggtagttttcaatctttgctcccctccttctctcctggctctagtagtccccagtgtctgctgttcccatcttttttttttttttttttttttttagacagagtctctgtcacccaggctggagtgcagtggcgcaatctcggctcactgcaacctccgccttccaggttcaagtgattcccctgcttcagcctcctgagtagctgggattacaggcgcctgctaccacgcccggctaattttttgtatttttagtggagacggggtttcaccatattagccaggatggtcttgatctccggacctcatgatccgcccgccttggcctcccaaagtgctgggatgacaggcgtgagccaccgcgactggcctcttcccaactttatgtccatgtgtacccaatgtttagctcccactttttaatttttttgagacaggacttgctctgtcacctaggacagagagcagttgtgcgatctctgctcactgcaacctcctcttctcaggttcaagcgattcttgtgcctcagccatcagagtagctgggattacaggcatgcaccaccatgcctggctaattcttgtattttttatagagaccagatttaatcatgttgcccaggctggactcaaactcctggcctcatttgatctgcccaccttggcctcctaaaagtgctgagattataggagtgagccaccgtgctcagcctagcttccacttacaagagaacatgagttattccaaactttgtaatcttaggataagtcccacttagtcataatgtataatcctttttctatgttgctggatttggtttactagtattttgttgaagattttttccgtttgtattcccaagagattattggtctgctatttgcttttcttgtgacatctttgtctggttttggtatcagggtattaagagtgacctcataaagttgaggacactcttctcaattgaggagtattttcttctcttctattttttaggagactctatgaaatattggtgttaattccttaccatctggcttacaatctggtcctgggcttttccctgtgggaagttttaaaagaattattattagtccaacctctttacttgtatatttcttcattaatacagaaattaacaaaatttgttactgatttctgattttattccaacatggtcagagaacatatgtagtataatttcaattcttttaaatttactgagacttgttttatggcctagcatgtgatctaccccagagaatgttccatgtgcacttgagaaggatgtgtattttgctgctgttgggtggagtgccttgtagatatttgtcaagtctagttggtttatagtgttttctattttcttgttgatcttctgcctagttgctctagctattattgaaatggagttttgagggttccaactattgtagttaaattgtctgtttcttccttcaattctctaagtttttatgtcatgtatctttaggctgtattgctaggtacatatgtttataattgtcatattttcctaatggactgacccttttatcaatataaaatgtccttggcatacaagtggccaagaaacatatgagacaatgttcatcatcactaatcaacagagaaatggaaatcacaaccacaataagatatcatctcacgccagtcagaatagctatattaaaaagtcaaaaaataacagatgctgaagaggctaaggaaaaaaagagaatgcttatacactgctggcaggaatgtaaattggttgaaccactgtggaaagaagtttggagatttctcaaagaatttaaaacagagcagctgggcatggtggctcatgcctgtaatcccagcactttgggaggctgaggcaggtcgatcacctgaggtcaggagttcaagaccagcctagccaacatggtgaaaccctgtctctgctaaaaatacagaaattagctgggcatggcggcacacgcctgtagtcccagctacttgggaggctgaggcaggagaatcgcttaaacccaggaggcggaggttgcagtgagcacagatcacaccactgcactccagcctgggtgacagagagagactccaccaaacaaacaaacaaacaaacaaaaacagagctaccattcaacatagcctcccattactgggtatatatccaaaagaaaacaattcattctaccagaaagacacatgcacctatatgtttatcacagtgctattcacaagagcaaagacatggaatcaacctaggtgcccatcaacagtggattggataaagaaaatatagtacatatataccatggaatactatgcagccataaaaaagaatgaaatcatgtcctttgcagtaacatggatgctgctggaggccattatcctaagtgaaataacacaggaacagaaaaccaaatattgcacagtctcataagtgggagccaaacattagatacacatggacacaaaaatggcaacaagagacactaaagatgacaagagggagaagggagggaggggtgcaaggattggaaagctaaccattaggtactatgcttactacttgggtaatgggatctgtaccccaacctcaggacccatgtaacaaacctgtgtatgtacctccagaatttaaaataaaagttggaactattaaaaaaaagtccttctttgtctatagaaacaatttttttcttaaagtttatgttgtctaacattagtatagctactccacttctctttgagttactgtttgcatggtatatctttttccatcattttactttcaacctgtttgtgtttttgaatctaaagtgtgttttgccaggtgcattggctgatgcctgtaatcccagctgcttaggggagactgaggcaggaggattgcctgaggacgggagttcaagaccagcttgggaaacacagtacgaccctatctctaaaaaaaaaaaaattttttttggagagatatctgcactcccatgtttactgcagccttgtttgcaatagccaagatttggaagcgacctaagtgtccatcagcagatgaatggataaagaaaatatattgcttatacacaatggagtactgttcagccataaagagtgagatcctgtcacttccaacaacatggatggaactgaagatcgttatgtgaagtgaaattagccaggtaagttttgaagtaagccaggtcctatctctaaaaaaattgttttaaattagccaagtatggtggcaggcacctatagttccagctacttgggtggctaaggtgggaagattacttgaaaccagaagtttgaggctgcagtgagctatcattacaccactagactccaacctaggcaacagagcaagactctgtctctaaataataaaaataaaaataaaatgaagtgtgttttttgtagatagcatatagttggatcatgatttttaaaaaaaatcaatttgccaatctctaccttctgattggagtatttaattcatttgcatttaatgaaattactgataaggcaggatttatctaccattttactgttggtttctttaggcctcttgccttttttttctcctctatttttcattacttccttctcttttcttatatattttctagtgtaacatttctgtttccttgtcattttttactatatatttaaaattatttacttagtggctggtgtgtcttgaggtggactctttgagtctttcctgcttagaatttgttgagcttcttggattcactttaatgtttttcctcaaagtgggaaaggttttggccactatttcttccagtatatgttttatccccttccctctctctcacttatctattctaggactcctattatgtgtatgttggtatgtttgatggtgtctgacgggtgtctgaagcactgatcatttttctttgctgattttttttttctgttccacagactggataatctcaaatgacttctaatttgctgattacttcttttaccagttcacacattttttaaacttctcaagtaaatctttcatttgcatttttgtactttgcaactctaaaatttctacttggttctattttataaactaactttctttccttttttcttttctttcttctttctcttttttctttctcaatctttctcttttcttccctccctcctttccctccctccctccctttctccttctttctgcctgcctttctttcctttctctttcttcctctctctttctccccttcctacctttcctccctccctctttccctccttctgcctctgtcctctctgtttgtgcagacacttaaggtcagacgaaagagctggggaattctcaggtctcttctgggcatgtgcacagtcctacacatgtgtgtggccttctgcattcttaggaataggttgaagcttttcaaaacgtcctatagaaatctcattcccagtttttccttctaagtcttttggtcagtttgtttgttccaactgttacagccaccttaggaagctgagatgttcaacaattgctgttgattttttttgacaaatgcacccagggaaaaggttgttcacactgggtaacctcttagtcacatcaaataaagacaagacctaggagtagggacttacatggaactaccaaaaaggccaaatggcaattctctggtaatgaagctttggaggagttccaatccccttctgagccctacggtggctgctctgctgctggatgtcagcatgattgtgtggccgaggctgttgtggagctggggaaagggggagtgggaatagggtacattaaaatgtcagaaagcttgcttttcttacccagatgcaaccctttccttttttttttttttttttttttgagacagagtctcgcactgtcacccaggctggatggagtgcagtggcgtgatctcggctcactgcaagctctgcctcctaggttcacgccattctcctgcctcagcctcccaagtagctgggactacaggcacctgccaccgcgcccggctaattttttgtatttttagtagagatggggtttcactgtgttagccaggatggtctccatctcctgacctcgtgatcgcccgccttggcctcccgaagtgctgggattacaggccttttcttgaataaatggattgctgcaagcctctggttaatgtctagacagttttgctagtgttctcattgcttttatggaagagagggttttcagaggttgttactctattatgcccactgatgtcctctcataatttttgaaaggaattatgcttgcaacaatcttcaagttctgctactatgtattgcattggagaggggttcattttcctttgccttcagggactgctatggtttgaatgtgttccccaaagtaaatgtgttggaaacttaatctctactgcaatagtgttgagaggtgggacctgtaagaggttaggtcacgagagctctaccctcatgaataaattaatgatgttatgccaggagtgggttagttatcacaggaatgggttgctagttaaagggtgagttagactccattcctctcttgccatgtgatgccttctgccatgctgaggcagcaagaaggccctcaccagatatagccccttgatattggacttctcatcctccagaaccgtgagccacatacacttctctgtaacattctgttatggcaatacaaaatagactaagatatggagggatgctttggggaaaacacttctaaaatatgggttatgggagaacttcaggttaagaaggaggtgtagctactgacaggaagtgggaccagtctttaagagaagtcttccaaaggctttgggcctgtccactctcagggtcctaagtaggtgcctgcctggatccatgtctgcttgcaccctgcaccctgcaccctgcccatgcaatctctgctgagtccactgggaatgtgtcatagtgtatgtgaaacctgtttggagtggagtgcctacacagggcttctggcatggaaacctcctctgtgccagaggtatatttatgaagtggaagcagccacagaaggcaggccagccatacaaaggaaagatgtccaaagcattcagccttattgcacaagaagttacaagttaataacaatttgcattaatgaaactctttctatccacaagactaagcatctcaggtgtgtgaggtttataggtatttaaaaacctggccttggtgaaatgctttacaagaactcgatacacaagacacgtaagaaacgatgggctgggactttggcagctgaaatagtctcagtgcttcactgagaagctcatcagttttgaaggacaatctgttggcttatgtattgggtaacatcctggggtcagcaaattactgcacatctggcctgcttttatacggcctatgagctaagagttggagaaaaaaacaaaaagtatgcaaaaaaggccctacatggtttgcaaagcctagcagatttattatctggccttttacagaaagtctgtctacccctgagtaacggcatcatggatttatatttactttattatttatttacttttgagacagggtcttgctctgttgctcaagctagagtacagtggtgtgaacatggttcactgcagcctcacacctcagcctcaagcgatcctcccacctcagccaccaccacatgccaccatgcccggctaattatatggtgaatttaaatgaccagtgatatcccaggacagtcaatacctacaacaagaaccaaagagcacaaaaacacttgaaatatcattactttactttagtgttccaggcattttaaatattcatacaatcgccttatttcagcagtcatttcctctccagtacagattttgtgtccagaaccagagccatgtacgtcactgaattttctctacagcacccgcatgctacacgggacctactccggtgcccatgtctttgctagtagagcctctcaccacacttgcaagagggctggacctccccttgcttgatgtagcctccactgtgaatgaaaacacactttgtcacttcgatcacagtacatttccagcactcccaggtgttccatgtatgtggcaatcatcccacagagctagtgacacatcatgtcagctggtacctatgtcagcacctgctccactatatcatacagatgctgaggcacttaaatgttcttggtaaaatggagttcataattgccataggagttgagttttggggaaagggactttcaataattaatacccttaatacatatttagcagatttataatttcgtgtctgtttacatttgttgtcaaagcttcataaactatttatgtaaatgaaagcatgtttgagtttccaaatgctgctatgacaagcaaacagagaaactgcttagacaacacctgcttgtgccataaatacatacggcaacatccggtcatccttaaagaaatgcttgtgtttccaaaaagaatttttttttttaagtcataagccttatgcaattcttccaagataataatgtgtttgtccttccttctcaagcatggttcaaggcatctcaaggcatattgctgtctgaggttctgatttaactgtccgggggtacaggggaagagtgggcactaacattttttaaaagcttcacagtcattccagcatgtagtcagtgttgagaaccttggtactaaaggctcttgcatcttcctactgtcacttgtcctcatcaaaagcccttgaggtagtccctgggtcaggcaatgatctctttcatgggctaagaaactaaggcacagagaggttaacaggctcctctgatactgtgcagtcaaatgacagaaccatgattgcaactgacatttccaaataaaccatgactcctcccccagcaacgggtagcacttacatggaccaaaagtatgaagcctgactgggagccaggcataaccttctgtgtcaaggacatcatggaagggaaaggaacagttctgaaccaatcattccgcatgaacagaaataaatacataaagccaggcttggtggtgtgcacctgtagtctcagctactcaggaggctgagacgggaggactgctcaagcccagaaattcgaggctgcagtgtgctatgattacaactgcgaatagccactgcaatccagcctgggcaacacagtgagaccacgtctctgtaaaattttatttaaaatttatttaaaatttatttaaatttatttgaaatttaaaatcaaattttaaaaatttaaaaaatattttttaaaaaggaaataagttcctaagatacttattggaagccacatgaggaatgaggcataactttttcttttcttaaaagtcttacttccctcttatatatgccattgagtcaggtttctcagaaaatccatcaagattcacagacttcctgacatctgaattcttagctctgttactgtgagggctagaaaactcgtgaatgtctctataatttgggtccaaaagataattacaaacctctgttagcatgtgacagcaatacaaaaatgcccatgctttccctgtcacccgcccacctagacttgccagggacccagaaccctacacgttctaactgggtatacatcttcccaggatccgatcagatctcactcccatctcagaatttcccaaacaccaacccatcggctgcgttgggcctcaaggattaatgactacaactgactgttttattttgctctacaggcaaacttttaaatctgtattctgggtaacccccaggacgtttattttgtaattccaaatttccatgagagccaattcacctgggaccttctccacttcaccccaaggtaacaccctcacatcctatcaactattgctgtacctaagaaataatttctatcattattgcctttttcattgtaagttctcacatctcatcatgttcaaggaggcattgattttctcctcttttgtaaaagtctcacctgactgcagaaatgttttcttgagccaagtagaaatgaggaatggagcacacataggcatgaagaaagaacgtagcacgttctggtggggagggcagttttcaatgggttgctgtgatttccaggacactctaggaagggcctgtttactcagcttacactgaacacaaatgacatcttgttctccctactgctagtgatgtggcctcctgaaaagcctataaagtattagttaatccagtaagcggaagccacttctaacagtacacatttgttgagatttacaagacactgtgtggagatgaaaccacttctttcccattttagaagacttccccattcaggcaggatatatactctcctaatacccacaggcacaggaactcgaatccttcctggaaggaaacctgtccctctagctactgcagaaagtgcttgggggcataaaaagaacaaaaagggggaaagcaacctttgtctggggcagggccacttggggagtggaattttactgactcctcatcctcaaagaggtttttacaaacgtttaaaaaaaagtaaaaaaagaaaaaaaaagggaactaggcaaaactgcatttagaattttggttaaagcaaagaaaattgagaaaattgaatcatcatattttcaaagacctaccatattcaacctattaagtaaagcaatatatcatgtttttttctctctcatgcttatttgatgcttacaggttcagggcagacttgccactttgtttctaaaacatgcagagagcagacttagagcagcatatgctgttttggggcccaacccgcacaaaccctgacaggtgactgaccaaacaccatcaggaaggtgatgagggaaaccacctttgccgagaggccagtgcacagcacaaaactaaggactgttggtgcatgcttgtacagagcttagtgtggcagagtgttaccgaagggatgggtggggaacacacaggcaacctccaatatgctctgacgtccaatccatagtccagagcagtggggctgcagccgggcatggagctaaggcactagggctgcagtgggtgggaggcaccgaccagaggtcccagtgccctgccgttcccggggagaggggaaggagctctgctcacaaagctgcctttgtgtaccaaagttgttttcaaaagtctcaacagcactgctgagagctacatctgggaagccccctgagcagccctctctttgggagctgcctcctctgctcacgtgccttcttccatctcatctttgcgagttgcctttctttcccctgctgtgggctggataaagagcaatccagtcatttcaccattccctggagcaggaccccgtgctttttccaaggcagcagggagtgccctctgtcacagcttgatgaaggcagctggctgggtctgaggttgctccacatctgggggtgggaagacactggaaatggctatgtccacgatgccttggcacagttctgcatagagcttctgagcacatgcaggggcaccgttgacctcaatgagccacaccttcagctcctcatcgaccatgaagtcaaagccgaagagctggaagctctggtaagggaggtgcttggtgctaatggcaggctccacgctcaggaggcagttccttattatatgtttgatttgtagtaagatactactttctagggtaatgttcaaagcacttgttaggtactgattgaactccttgaagaacatttcatttccttcttcatacttcccgtagttctttgaatactctttttgaatgcagtgattggtcaaatggcaggttttgtcttggaaattatcaacatgatatggttctgaagcagtccgaagcacaccctctctatagaggtagatattatactgatgatccaccaagacccagcttcggatgtcaaacttgcgatgacctggctcaagcagcagagggtgctcaagatatttctggatcacgtgcacttggccctggttgtctatgaaatcgagaagctctgaagcctctgaggagatgagaatgccttcacctttggcaccggctgatgactttgcaatccaaacgttgccctctccatcctctttctttctgttataagaggcgagaaagaattctctttcatctgtccttgagttactgattggtggctgaattccattctgtgctggagcaactggagtcttgagattggttggataaatcacataagattcagggaaccatgtgcaggactcagccagttcagggcttgtcttgattagcttcactaaagaagctttgcgacacagtttgtcagcacccctgtagtaattcaccaactgtaccagcccgggctcgtgacccagtctcccgaagggcagccgattcctctctcccagcatcaggttgaatctggggttgtctcgccgcagcctcttccagtggccggtggcgaggagcagccgggagacctcggcgtagacgctgctgttctcatcgcgtaccacgaaggtgtacatggcgaagcgccgcgcgcccgggccgccgggcagccgccgcagggaccaggcggccgagaaggcggctcagcgcggaccccgcccgggcgcccgccgcggcccggcccccgccgcccgcgccggctaccgcgcctctcgggtgccggcggcgccgcgcccgggcgcccgccgggtgccggagaggaaagc

SEQ ID NO: 14431 - RNA, 4468 nt, Homo sapiens
  source 1..4468: mol_type = other RNA
gctgggattacaggcatgagccaccgcgcgcgcccggccaactgagtagttgtagttctttatatagcctatactagtccttgtcagatccatgatttgcaaatatttttctcccattctgtgggtttttactttcttgctggtgtcctttgaagcaaaacgttttaattttgaagtgtagtttttttcttttgttgcctgtctttttatatcatatctaagacatcattgtgtaatccaaggtcatgaggatttaaaaaaaaatttatgggtacataattagcatatttatgaggtatatgagatgttttcatataggcatacgatgtaatcatcacaggagggtagatggggtttccatcacctcaagcattcatcatttctgtcatgaacattccaattgtacttcctcagttatttttgaaggtacaacaaattattgctgactgcagtcaccctgttgtgctatcaaatactagatatttttcaatcatggggattttcacctatattttctactaagagttttgtagtttcaactcttacatttaagtctttgactcattctgagctaatttttgtatatggtgtgagaaaggcatatcactttattcctttgcatgtggatatccagttgtcctaacaccatttgttaaaaagactattctttccctcatcaaattgtcttggcctccttgtcgaaaatcagttcactatagatgcaagggtttatttttgactctcagttctattctcttgatctgtatgtctatctacatttatctgtatatctgtctacaaactacacagatttgattaatacagctttgtaataaattttgaaatcaggaagtgcacatcctccaactttgttcttctttctccagatttatttgatcctttgtatttcaatatggattttagcgtcagcttagcttgtcaatttctttctcttttttttttttttttgttttttgtttttttgagacagagttttgctcttgttgctgaggatggagtgcagtggcatgatcttggctcactgcaacctctacctcctgcctcagcctcccaaatagctgagattacaggcatgcaccaccatgcctggctaattttgtatttttaatagagacagggttttaccatgttggccaagctggtcttgaattcctgacctcaagtaatccatctgccttggccgcccaaagtgctgggattacaggtgtgagccaccacacccggcccagcttgtcaatttctgcaaagaaggctgagattcttgatcaggattgtgttcaattggtagatcaatttggggcctattttcatcctaacaataattatctcccaatccataaacatgggatgtctttccatttatttaggtgttctttaatttctttcagagatgttttgtagtatttggtgtagaaatgaacttttgttaaatttattcctaagtatttcattctttttggtgttgatataaatggaattgttttcttaacttcaaattgtttgtaatatgtagaaataccattgagttttgtatattgatcttgtgtctggcaatcttgctaaactctttattagttctaacagcgtaagtggatttcttaggactttttctatatggtatcttgtcgtctgcaaagagagatcatcatacttctccctttccaatctgaatgcgcagtcttctttccttccttttgtcgaattgctctgtctagaacatttaatacaatgttgaagtgacaagaataaatatacttgttttgtgcctgatattgggaagaaagctcccaactggagctttcacatcaccattaatatgatgtaggctgtgggtttttccaaagatgctctttatcatgttgaggaagtaatttatttctagtttgttgaaaggttttttccaagaaagagtgttgtgtattgccaaatgctttttcagtgtatattgaaatgatcatgtgctttttgtcctcttttttctattaaagtggtatattatattaagtaaattttgtatgttaaaaaaaccttgcattctttcttttccccttctcaacgtttattttagaatcaggggggtacatgtgcgaatttgttacaaaggtatattgggtgatgctgaggtctggggtatggttgaacctgtcacccaggtagcgagcacagtatccaataggtagttttcaatctttgctcccctccttctctcctggctctagtagtccccagtgtctgctgttcccatcttttttttttttttttttttttttagacagagtctctgtcacccaggctggagtgcagtggcgcaatctcggctcactgcaacctccgccttccaggttcaagtgattcccctgcttcagcctcctgagtagctgggattacaggcgcctgctaccacgcccggctaattttttgtatttttagtggagacggggtttcaccatattagccaggatggtcttgatctccggacctcatgatccgcccgccttggcctcccaaagtgctgggatgacaggcgtgagccaccgcgactggcctcttcccaactttatgtccatgtgtacccaatgtttagctcccactttttaatttttttgagacaggacttgctctgtcacctaggacagagagcagttgtgcgatctctgctcactgcaacctcctcttctcaggttcaagcgattcttgtgcctcagccatcagagtagctgggattacaggcatgcaccaccatgcctggctaattcttgtattttttatagagaccagatttaatcatgttgcccaggctggactcaaactcctggcctcatttgatctgcccaccttggcctcctaaaagtgctgagattataggagtgagccaccgtgctcagcctagcttccacttacaagagaacatgagttattccaaactttgtaatcttaggataagtcccacttagtcataatgtataatcctttttctatgttgctggatttggtttactagtattttgttgaagattttttccgtttgtattcccaagagattattggtctgctatttgcttttcttgtgacatctttgtctggttttggtatcagggtattaagagtgacctcataaagttgaggacactcttctcaattgaggagtattttcttctcttctattttttaggagactctatgaaatattggtgttaattccttaccatctggcttacaatctggtcctgggcttttcctgagcacatgcaggggcaccgttgacctcaatgagccacaccttcagctcctcatcgaccatgaagtcaaagccgaagagctggaagctctggtaagggaggtgcttggtgctaatggcaggctccacgctcaggaggcagttccttattatatgtttgatttgtagtaagatactactttctagggtaatgttcaaagcacttgttaggtactgattgaactccttgaagaacatttcatttccttcttcatacttcccgtagttctttgaatactctttttgaatgcagtgattggtcaaatggcaggttttgtcttggaaattatcaacatgatatggttctgaagcagtccgaagcacaccctctctatagaggtagatattatactgatgatccaccaagacccagcttcggatgtcaaacttgcgatgacctggctcaagcagcagagggtgctcaagatatttctggatcacgtgcacttggccctggttgtctatgaaatcgagaagctctgaagcctctgaggagatgagaatgccttcacctttggcaccggctgatgactttgcaatccaaacgttgccctctccatcctctttctttctgttataagaggcgagaaagaattctctttcatctgtccttgagttactgattggtggctgaattccattctgtgctggagcaactggagtcttgagattggttggataaatcacataagattcagggaaccatgtgcaggactcagccagttcagggcttgtcttgattagcttcactaaagaagctttgcgacacagtttgtcagcacccctgtagtaattcaccaactgtaccagcccgggctcgtgacccagtctcccgaagggcagccgattcctctctcccagcatcaggttgaatctggggttgtctcgccgcagcctcttccagtggccggtggcgaggagcagccgggagacctcggcgtagacgctgctgttctcatcgcgtaccacgaaggtgtacatggcgaagcgccgcgcgcccgggccgccgggcagccgccgcagggaccaggcggccgagaaggcggctcagcgcggaccccgcccgggcgcccgccgcggcccggcccccgccgcccgcgccggctaccgcgcctctcgggtgccggcggcgccgcgcccgggcgcccgccgggtgccggagaggaaagc

SEQ ID NO: 14432 - RNA, 2761 nt, Homo sapiens
  source 1..2761: mol_type = other RNA
gctgggattacaggcatgagccaccgcggccagccataactctgtgactcttgttacaaaggccttatattttgctctttgagggtggttttggtttgatgcctgttggttgccatcttttaactagggatgttttatcaaaatgcccagccaaagtgtccaaacaaattataccttaaagtttgaaaatgtctggcacttctaattcaatgcctgttgtgccaggcactgggctgctgaggaactgagtcccgtccctgcaggctagctagagaacacacacacacacacacacacacacacacacacacacacacacacacacacagagtggtcttacaagtcagttttatattctacctatatgcaataaaggtattattatgttgaggtgccttgatataaaaatttttcttaaaggagaggatgcctaaaacaggcattacctgaaacctcctctctccagcattggttgtcttctgtcatgactcagggttttcactgagaatgggatggaaatgtggtctaaagatagggccaatgttgggactggatcccctctgggaagtcagaccaggctagggcaggtccttgaagccatcaggaaaagcctctctgggaggcttatttgctttgagaacatatgtcctgcagttttgttcatatggcagtgaagtttcgtgcacacactctagagccaggcagcctgggttcaaagcgcagctctgccaggtcctaactgcatgaatttgggcaagtcgctcaacctctccatgcctgagtttcctcatcattagcagggatgacagggagtgcaggagtgcggtcgactcccagatattggagagcgctgggctagctgcccattctcccggcctccactcctctttgctgtccagccatcacttgctctttgaaggcaaacaaaacagaaaacagtgccaaaagtatgggaagaaagccagcttctcccctggggtgcctgtgatgccatgcccaccctccctgaccacgcagcccctgtggaccctcagggccccaagcccccatttccatcacatgcgtacacccatgtgtgtccatagccgcccatctcagtcaataaggctgctcctgcccacttggaatagtggtgacaaccaggagtggcttatgggaactatcccaatggcctgacagcatgtccgctgcaaaccgctgaggtaggacactgccctcatgtctagctgatcagcaagaggcgcagttgctttcttaggtaacattgctgctgtgtcctggccattgctggggggtggcacttaatctacaccagatttttccctcctgtatcttccgagctgcttggatcttggtgctgaattaggttggactttgtcttgtggggaagggaggactatagaccctcaacgtaagcaatggtcagactattctaagaaaactcgccgaattaaagcatgaggtaaatttagttctgacttctgtccaccccactgccactgtccccttttatcccatgatcccttgcttttcttttcctcctctctccctatctcttgtgtttgacgcatgataggaattcagaaatatatgtttgtggatttgtttattcacgtagcaaaccatttcttgagtgcctaccatgggccaggtagaatgggcggccccgggctgcagtggtttcttcagcccctctcctgggtttacactgtgcaagacggtttgtgatgggtcctcccatcgaggaccacactcttctttctctgtgccccttggtcctcagtctctgaccccacttcaaaggcagcattcactcagggaagctcccatacaatgctagtcagagtaaaagtttggacaaattgccaggaagcagcttgtcagtatgcataaacagcctttaaaatattactactctttgacccagaatttcacttctaggaatctgtcctaaggaagtagtcacatgcaaaagatttatgtaccaagatgttcatcaaagtgttgtttataacaggaagtctcagaagctggataaatatccaacctctggaaatggttagatagaatagtatgtagccattagaaaattatgtctatggggtttaaaatgtcatgggaaaacacttctgacataaaagagcatgagaactgtatatttagcataatcttaactatgttttagaatgcacaggaaaaaaatgtacaaacatattcatagtgatgtctctggtggtaggattatgatcagtaagtacttctgtctcttcatattttcctgtatttgataatacatgcatatgttgtttttaaaataagaaaaattttaagtttaaaattggagctgaaaagtgtttttaggtcaggcgaggtggctcacacctgtaatagcaccactttgggaggctgaggcagtcagatcacttgagcccaggagttcgagaccagcctggccaacatggtgaaaccccatctctactaaaaataaaaaaattagccatgtgtggtggcacacatctgtaatcccagctacttgggaggctgaggcatgagaattgcttgaacccaggaggtggaggttgcagtgagccaagatcgtgccactgcactctagtctgggcaacagagtaagactctatgtcaaagaaaaaaaaaaaagaaaagcctttttaaacagtagcagacataactatataatccttactaagctgtcggtcaaatttttatttatatatttattttattcatttattatttttag

SEQ ID NO: 14433 - RNA, 2787 nt, Homo sapiens
  source 1..2787: mol_type = other RNA
gctgggattacaggcatgagccaccgcggccagccataactctgtgactcttgttacaaaggccttatattttgctctttgagggtggttttggtttgatgcctgttggttgccatcttttaactagggatgttttatcaaaatgcccagccaaagtgtccaaacaaattataccttaaagtttgaaaatgtctggcacttctaattcaatgcctgttgtgccaggcactgggctgctgaggaactgagtcccgtccctgcaggctagctagagaacacacacacacacacacacacacacacacacacacacacacacacacacacagagtggtcttacaagtcagttttatattctacctatatgcaataaaggtattattatgttgaggtgccttgatataaaaatttttcttaaaggagaggatgcctaaaacaggcattacctgaaacctcctctctccagcattggttgtcttctgtcatgactcagggttttcactgagaatgggatggaaatgtggtctaaagatagggccaatgttgggactggatcccctctgggaagtcagaccaggctagggcaggtccttgaagccatcaggaaaagcctctctgggaggcttatttgctttgagaacatatgtcctgcagttttgttcatatggcagtgaagtttcgtgcacacactctagagccaggcagcctgggttcaaagcgcagctctgccaggtcctaactgcatgaatttgggcaagtcgctcaacctctccatgcctgagtttcctcatctgtaagattggagcaatggtaataccattagcagggatgacagggagtgcaggagtgcggtcgactcccagatattggagagcgctgggctagctgcccattctcccggcctccactcctctttgctgtccagccatcacttgctctttgaaggcaaacaaaacagaaaacagtgccaaaagtatgggaagaaagccagcttctcccctggggtgcctgtgatgccatgcccaccctccctgaccacgcagcccctgtggaccctcagggccccaagcccccatttccatcacatgcgtacacccatgtgtgtccatagccgcccatctcagtcaataaggctgctcctgcccacttggaatagtggtgacaaccaggagtggcttatgggaactatcccaatggcctgacagcatgtccgctgcaaaccgctgaggtaggacactgccctcatgtctagctgatcagcaagaggcgcagttgctttcttaggtaacattgctgctgtgtcctggccattgctggggggtggcacttaatctacaccagatttttccctcctgtatcttccgagctgcttggatcttggtgctgaattaggttggactttgtcttgtggggaagggaggactatagaccctcaacgtaagcaatggtcagactattctaagaaaactcgccgaattaaagcatgaggtaaatttagttctgacttctgtccaccccactgccactgtccccttttatcccatgatcccttgcttttcttttcctcctctctccctatctcttgtgtttgacgcatgataggaattcagaaatatatgtttgtggatttgtttattcacgtagcaaaccatttcttgagtgcctaccatgggccaggtagaatgggcggccccgggctgcagtggtttcttcagcccctctcctgggtttacactgtgcaagacggtttgtgatgggtcctcccatcgaggaccacactcttctttctctgtgccccttggtcctcagtctctgaccccacttcaaaggcagcattcactcagggaagctcccatacaatgctagtcagagtaaaagtttggacaaattgccaggaagcagcttgtcagtatgcataaacagcctttaaaatattactactctttgacccagaatttcacttctaggaatctgtcctaaggaagtagtcacatgcaaaagatttatgtaccaagatgttcatcaaagtgttgtttataacaggaagtctcagaagctggataaatatccaacctctggaaatggttagatagaatagtatgtagccattagaaaattatgtctatggggtttaaaatgtcatgggaaaacacttctgacataaaagagcatgagaactgtatatttagcataatcttaactatgttttagaatgcacaggaaaaaaatgtacaaacatattcatagtgatgtctctggtggtaggattatgatcagtaagtacttctgtctcttcatattttcctgtatttgataatacatgcatatgttgtttttaaaataagaaaaattttaagtttaaaattggagctgaaaagtgtttttaggtcaggcgaggtggctcacacctgtaatagcaccactttgggaggctgaggcagtcagatcacttgagcccaggagttcgagaccagcctggccaacatggtgaaaccccatctctactaaaaataaaaaaattagccatgtgtggtggcacacatctgtaatcccagctacttgggaggctgaggcatgagaattgcttgaacccaggaggtggaggttgcagtgagccaagatcgtgccactgcactctagtctgggcaacagagtaagactctatgtcaaagaaaaaaaaaaaagaaaagcctttttaaacagtagcagacataactatataatccttactaagctgtcggtcaaatttttatttatatatttattttattcatttattatttttag

SEQ ID NO: 14434 - RNA, 2790 nt, Homo sapiens
  source 1..2790: mol_type = other RNA
gctgggattacaggcatgagccaccgcggccagccataactctgtgactcttgttacaaaggccttatattttgctctttgagggtggttttggtttgatgcctgttggttgccatcttttaactagggatgttttatcaaaatgcccagccaaagtgtccaaacaaattataccttaaagtttgaaaatgtctggcacttctaattcaatgcctgttgtgccaggcactgggctgctgaggaactgagtcccgtccctgcaggctagctagagaacacacacacacacacacacacacacacacacacacacacacacacacacacagagtggtcttacaagtcagttttatattctacctatatgcaataaaggtattattatgttgaggtgccttgatataaaaatttttcttaaaggagaggatgcctaaaacaggcattacctgaaacctcctctctccagcattggttgtcttctgtcatgactcagggttttcactgagaatgggatggaaatgtggtctaaagatagggccaatgttgggactggatcccctctgggaagtcagaccaggctagggcaggtccttgaagccatcaggaaaagcctctctgggaggcttatttgctttgagaacatatgtcctgcagttttgttcatatggcagtgaagtttcgtgcacacactctagagccaggcagcctgggttcaaagcgcagctctgccaggtcctaactgcatgaatttgggcaagtcgctcaacctctccatgcctgagtttcctcatctgtaagattggagcaatggtaatacctgcattagcagggatgacagggagtgcaggagtgcggtcgactcccagatattggagagcgctgggctagctgcccattctcccggcctccactcctctttgctgtccagccatcacttgctctttgaaggcaaacaaaacagaaaacagtgccaaaagtatgggaagaaagccagcttctcccctggggtgcctgtgatgccatgcccaccctccctgaccacgcagcccctgtggaccctcagggccccaagcccccatttccatcacatgcgtacacccatgtgtgtccatagccgcccatctcagtcaataaggctgctcctgcccacttggaatagtggtgacaaccaggagtggcttatgggaactatcccaatggcctgacagcatgtccgctgcaaaccgctgaggtaggacactgccctcatgtctagctgatcagcaagaggcgcagttgctttcttaggtaacattgctgctgtgtcctggccattgctggggggtggcacttaatctacaccagatttttccctcctgtatcttccgagctgcttggatcttggtgctgaattaggttggactttgtcttgtggggaagggaggactatagaccctcaacgtaagcaatggtcagactattctaagaaaactcgccgaattaaagcatgaggtaaatttagttctgacttctgtccaccccactgccactgtccccttttatcccatgatcccttgcttttcttttcctcctctctccctatctcttgtgtttgacgcatgataggaattcagaaatatatgtttgtggatttgtttattcacgtagcaaaccatttcttgagtgcctaccatgggccaggtagaatgggcggccccgggctgcagtggtttcttcagcccctctcctgggtttacactgtgcaagacggtttgtgatgggtcctcccatcgaggaccacactcttctttctctgtgccccttggtcctcagtctctgaccccacttcaaaggcagcattcactcagggaagctcccatacaatgctagtcagagtaaaagtttggacaaattgccaggaagcagcttgtcagtatgcataaacagcctttaaaatattactactctttgacccagaatttcacttctaggaatctgtcctaaggaagtagtcacatgcaaaagatttatgtaccaagatgttcatcaaagtgttgtttataacaggaagtctcagaagctggataaatatccaacctctggaaatggttagatagaatagtatgtagccattagaaaattatgtctatggggtttaaaatgtcatgggaaaacacttctgacataaaagagcatgagaactgtatatttagcataatcttaactatgttttagaatgcacaggaaaaaaatgtacaaacatattcatagtgatgtctctggtggtaggattatgatcagtaagtacttctgtctcttcatattttcctgtatttgataatacatgcatatgttgtttttaaaataagaaaaattttaagtttaaaattggagctgaaaagtgtttttaggtcaggcgaggtggctcacacctgtaatagcaccactttgggaggctgaggcagtcagatcacttgagcccaggagttcgagaccagcctggccaacatggtgaaaccccatctctactaaaaataaaaaaattagccatgtgtggtggcacacatctgtaatcccagctacttgggaggctgaggcatgagaattgcttgaacccaggaggtggaggttgcagtgagccaagatcgtgccactgcactctagtctgggcaacagagtaagactctatgtcaaagaaaaaaaaaaaagaaaagcctttttaaacagtagcagacataactatataatccttactaagctgtcggtcaaatttttatttatatatttattttattcatttattatttttag

SEQ ID NO: 14435 - RNA, 3532 nt, Homo sapiens
  source 1..3532: mol_type = other RNA
gctgggattacaggcatgagccaccgcggccagccataactctgtgactcttgttacaaaggccttatattttgctctttgagggtggttttggtttgatgcctgttggttgccatcttttaactagggatgttttatcaaaatgcccagccaaagtgtccaaacaaattataccttaaagtttgaaaatgtctggcacttctaattcaatgcctgttgtgccaggcactgggctgctgaggaactgagtcccgtccctgcaggctagctagagaacacacacacacacacacacacacacacacacacacacacacacacacacacagagtggtcttacaagtcagttttatattctacctatatgcaataaaggtattattatgttgaggtgccttgatataaaaatttttcttaaaggagaggatgcctaaaacaggcattacctgaaacctcctctctccagcattggttgtcttctgtcatgactcagggttttcactgagaatgggatggaaatgtggtctaaagatagggccaatgttgggactggatcccctctgggaagtcagaccaggctagggcaggtccttgaagccatcaggaaaagcctctctgggaggcttatttgctttgagaacatatgtcctgcagttttgttcatatggcagtgaagtttcgtgcacacactctagagccaggcagcctgggttcaaagcgcagctctgccaggtcctaactgcatgaatttgggcaagtcgctcaacctctccatgcctgagtttcctcatctgtaagattggagcaatggtaatacctgctttttagggttgagaagagaattaaatgaattaagatgggtaaagtgcttagagtggagctttgcaagtagtaagtgctatgtaagtgttcgatttaaaatgaaagacccttaaatacattctttgttcatttcacaagcccttcatttcacaaccttacatttcacaaccaagctctgtctcccctggaatccagccataactctgctcacaagtgtgagacaggccccagcagagctgcacgaagaggagagaaggcagccccccagactcccaaccccctgtccaagatggcaaaaccagaacacagcctctgtaccaccccagcaggtattcagaatctgcaatctccaaagcccacttcaattgtaaatgtagagccacgtgcgctttaagtcacctgtcactctggaggctcttttgctcagttcctcaccattagcagggatgacagggagtgcaggagtgcggtcgactcccagatattggagagcgctgggctagctgcccattctcccggcctccactcctctttgctgtccagccatcacttgctcttccccaccccctcggaactcagaggtggtgcaggaatttggactccaagaattaacagctccaccaccatcaccagagccaaaactcaggatgcatgtgcttcatctgctgcttatttccagctgagagccagtggtgccatggttccttagggagccggtcccctgatgccggctcctggccccaaatctctctgatccgggctcttccagaatgtcttgtctccaccatcgcctttgaccaatggtgtccctttgcctggtaatgtcccctttgcctgatgatggccctgtcactcctctctttagcacagaggaggctgtttcatcccttcaagcctgccctcccttcaagtcttagctcaagttcaccttctccgcagagccttctccaatcttcttgactacgtctcctctcggctccagcaacctctgtctctggcactgattccttacttagctaagagaatcacagacacttggggctcaggacaatctgctttctctcttcttacccatggccttggactgtgtgtacctctttgtctccactcccaaacccaacccccagagggcagagagcatgttgtctgtccctttgctcagcatgaagccatgcgtgtggtagatcggcagagttccataacttgtgttgaccgaggggtcactttgctctgaaattacccctgtgtccttcagtatttgcacagatagcttcctggccagaccgaatatatccaagggcatggcccacctctgctcctgtttccaggtccctggtgggggttagttcatgccttcctcataatctgcccactggcctggtcctcaaggtcttcccaactgctcagccagagttgagaaaatgggtcgctccatcctgtttgtgtcgttctctccttcctggcccactctcctgcccacaggtatccaggggctgcctgtagcattagaggacatacatgcacatgcgtgggcatgggacactcacgtagcctccaagcacagcatcaataatgcattctgtgctttatagcatggaaagctgctctaaactttattacacagtggacatgtctgaagcagctcccaaatccacccctgagtgtgttggaattggcaagcctatcacttgggagtctagtttttttgttcgttaataatagatgcttcctgtggccccagcttggcaattttgatttaaagtgatcttaactgaagagactaatggacgggtctgaatttgtgccttttaagcacaaagtattgctcttaattaactggattctatcctttgagcaggcagaggccttcccccaagggcgtcattaacgatccacatctggacatcttccaaagccttcttctgtttcaggccaaccgcaggtgtgttcctgaacacccaggaggctatgagagccacatatgcctcccaaatacacacagtgtgcatgcccagggacatagagcagtgtgcaaagtcccattccatctctctccacctgggagaggatggctcttctgtctgattcatggctcaaagtggtaaaggagctccccactccccgtcccacgcctactcagagtctgcaaatatgtatgcgatatgagagctcgtcagttagctgtcttcagtgtggcgcacatttgaggagtctgactcccctccagcacaggccaatgtgcactgctctcctatctttgtacccccactgttgcactgtgcagaggttggagccatagaagtaccagagctgtgaaaggagaggccccctctcacctctgccctggtctccatccccactttctctaggaagctagtaggtgctgacaggggagagaagggaggggaggggtccagaaacagtggctcatgcctgcaatcctagcactttgggaggctgaggcaggaggatcatttgaggtcaggagtttgagaccagcctgggcaatgtagcaagaccctatctctacaaaaagaaaaaatgtaattagctgggtgtggtggtgggcacctgtagtcctagctacttgggaggatgaggtgggaggattgcttgagcccaagagtttgaggttacagtaagctgtgattgcaccactgcactccagcctgggcaacagagctgagaccctatctcaaaaaaagaaaaa

SEQ ID NO: 14436 - RNA, 2823 nt, Homo sapiens
  source 1..2823: mol_type = other RNA
gctgggattacaggcatgagccaccgcggccagccataactctgtgactcttgttacaaaggccttatattttgctctttgagggtggttttggtttgatgcctgttggttgccatcttttaactagggatgttttatcaaaatgcccagccaaagtgtccaaacaaattataccttaaagtttgaaaatgtctggcacttctaattcaatgcctgttgtgccaggcactgggctgctgaggaactgagtcccgtccctgcaggctagctagagaacacacacacacacacacacacacacacacacacacacacacacacacacacagagtggtcttacaagtcagttttatattctacctatatgcaataaaggtattattatgttgaggtgccttgatataaaaatttttcttaaaggagaggatgcctaaaacaggcattacctgaaacctcctctctccagcattggttgtcttctgtcatgactcagggttttcactgagaatgggatggaaatgtggtctaaagatagggccaatgttgggactggatcccctctgggaagtcagaccaggctagggcaggtccttgaagccatcaggaaaagcctctctgggaggcttatttgctttgagaacatatgtcctgcagttttgttcatatggcagtgaagtttcgtgcacacactctagagccaggcagcctgggttcaaagcgcagctctgccaggtcctaactgcatgaatttgggcaagtcgctcaacctctccatgcctgagtttcctcatctgtaagattggagcaatggtaatacctgtcactctggaggctcttttgctcagttcctcaccattagcagggatgacagggagtgcaggagtgcggtcgactcccagatattggagagcgctgggctagctgcccattctcccggcctccactcctctttgctgtccagccatcacttgctctttgaaggcaaacaaaacagaaaacagtgccaaaagtatgggaagaaagccagcttctcccctggggtgcctgtgatgccatgcccaccctccctgaccacgcagcccctgtggaccctcagggccccaagcccccatttccatcacatgcgtacacccatgtgtgtccatagccgcccatctcagtcaataaggctgctcctgcccacttggaatagtggtgacaaccaggagtggcttatgggaactatcccaatggcctgacagcatgtccgctgcaaaccgctgaggtaggacactgccctcatgtctagctgatcagcaagaggcgcagttgctttcttaggtaacattgctgctgtgtcctggccattgctggggggtggcacttaatctacaccagatttttccctcctgtatcttccgagctgcttggatcttggtgctgaattaggttggactttgtcttgtggggaagggaggactatagaccctcaacgtaagcaatggtcagactattctaagaaaactcgccgaattaaagcatgaggtaaatttagttctgacttctgtccaccccactgccactgtccccttttatcccatgatcccttgcttttcttttcctcctctctccctatctcttgtgtttgacgcatgataggaattcagaaatatatgtttgtggatttgtttattcacgtagcaaaccatttcttgagtgcctaccatgggccaggtagaatgggcggccccgggctgcagtggtttcttcagcccctctcctgggtttacactgtgcaagacggtttgtgatgggtcctcccatcgaggaccacactcttctttctctgtgccccttggtcctcagtctctgaccccacttcaaaggcagcattcactcagggaagctcccatacaatgctagtcagagtaaaagtttggacaaattgccaggaagcagcttgtcagtatgcataaacagcctttaaaatattactactctttgacccagaatttcacttctaggaatctgtcctaaggaagtagtcacatgcaaaagatttatgtaccaagatgttcatcaaagtgttgtttataacaggaagtctcagaagctggataaatatccaacctctggaaatggttagatagaatagtatgtagccattagaaaattatgtctatggggtttaaaatgtcatgggaaaacacttctgacataaaagagcatgagaactgtatatttagcataatcttaactatgttttagaatgcacaggaaaaaaatgtacaaacatattcatagtgatgtctctggtggtaggattatgatcagtaagtacttctgtctcttcatattttcctgtatttgataatacatgcatatgttgtttttaaaataagaaaaattttaagtttaaaattggagctgaaaagtgtttttaggtcaggcgaggtggctcacacctgtaatagcaccactttgggaggctgaggcagtcagatcacttgagcccaggagttcgagaccagcctggccaacatggtgaaaccccatctctactaaaaataaaaaaattagccatgtgtggtggcacacatctgtaatcccagctacttgggaggctgaggcatgagaattgcttgaacccaggaggtggaggttgcagtgagccaagatcgtgccactgcactctagtctgggcaacagagtaagactctatgtcaaagaaaaaaaaaaaagaaaagcctttttaaacagtagcagacataactatataatccttactaagctgtcggtcaaatttttatttatatatttattttattcatttattatttttag

SEQ ID NO: 14437 - RNA, 2797 nt, Homo sapiens
  source 1..2797: mol_type = other RNA
gctgggattacaggcatgagccaccgcggccagccataactctgtgactcttgttacaaaggccttatattttgctctttgagggtggttttggtttgatgcctgttggttgccatcttttaactagggatgttttatcaaaatgcccagccaaagtgtccaaacaaattataccttaaagtttgaaaatgtctggcacttctaattcaatgcctgttgtgccaggcactgggctgctgaggaactgagtcccgtccctgcaggctagctagagaacacacacacacacacacacacacacacacacacacacacacacacacacacagagtggtcttacaagtcagttttatattctacctatatgcaataaaggtattattatgttgaggtgccttgatataaaaatttttcttaaaggagaggatgcctaaaacaggcattacctgaaacctcctctctccagcattggttgtcttctgtcatgactcagggttttcactgagaatgggatggaaatgtggtctaaagatagggccaatgttgggactggatcccctctgggaagtcagaccaggctagggcaggtccttgaagccatcaggaaaagcctctctgggaggcttatttgctttgagaacatatgtcctgcagttttgttcatatggcagtgaagtttcgtgcacacactctagagccaggcagcctgggttcaaagcgcagctctgccaggtcctaactgcatgaatttgggcaagtcgctcaacctctccatgcctgagtttcctcatctgtcactctggaggctcttttgctcagttcctcaccattagcagggatgacagggagtgcaggagtgcggtcgactcccagatattggagagcgctgggctagctgcccattctcccggcctccactcctctttgctgtccagccatcacttgctctttgaaggcaaacaaaacagaaaacagtgccaaaagtatgggaagaaagccagcttctcccctggggtgcctgtgatgccatgcccaccctccctgaccacgcagcccctgtggaccctcagggccccaagcccccatttccatcacatgcgtacacccatgtgtgtccatagccgcccatctcagtcaataaggctgctcctgcccacttggaatagtggtgacaaccaggagtggcttatgggaactatcccaatggcctgacagcatgtccgctgcaaaccgctgaggtaggacactgccctcatgtctagctgatcagcaagaggcgcagttgctttcttaggtaacattgctgctgtgtcctggccattgctggggggtggcacttaatctacaccagatttttccctcctgtatcttccgagctgcttggatcttggtgctgaattaggttggactttgtcttgtggggaagggaggactatagaccctcaacgtaagcaatggtcagactattctaagaaaactcgccgaattaaagcatgaggtaaatttagttctgacttctgtccaccccactgccactgtccccttttatcccatgatcccttgcttttcttttcctcctctctccctatctcttgtgtttgacgcatgataggaattcagaaatatatgtttgtggatttgtttattcacgtagcaaaccatttcttgagtgcctaccatgggccaggtagaatgggcggccccgggctgcagtggtttcttcagcccctctcctgggtttacactgtgcaagacggtttgtgatgggtcctcccatcgaggaccacactcttctttctctgtgccccttggtcctcagtctctgaccccacttcaaaggcagcattcactcagggaagctcccatacaatgctagtcagagtaaaagtttggacaaattgccaggaagcagcttgtcagtatgcataaacagcctttaaaatattactactctttgacccagaatttcacttctaggaatctgtcctaaggaagtagtcacatgcaaaagatttatgtaccaagatgttcatcaaagtgttgtttataacaggaagtctcagaagctggataaatatccaacctctggaaatggttagatagaatagtatgtagccattagaaaattatgtctatggggtttaaaatgtcatgggaaaacacttctgacataaaagagcatgagaactgtatatttagcataatcttaactatgttttagaatgcacaggaaaaaaatgtacaaacatattcatagtgatgtctctggtggtaggattatgatcagtaagtacttctgtctcttcatattttcctgtatttgataatacatgcatatgttgtttttaaaataagaaaaattttaagtttaaaattggagctgaaaagtgtttttaggtcaggcgaggtggctcacacctgtaatagcaccactttgggaggctgaggcagtcagatcacttgagcccaggagttcgagaccagcctggccaacatggtgaaaccccatctctactaaaaataaaaaaattagccatgtgtggtggcacacatctgtaatcccagctacttgggaggctgaggcatgagaattgcttgaacccaggaggtggaggttgcagtgagccaagatcgtgccactgcactctagtctgggcaacagagtaagactctatgtcaaagaaaaaaaaaaaagaaaagcctttttaaacagtagcagacataactatataatccttactaagctgtcggtcaaatttttatttatatatttattttattcatttattatttttag

SEQ ID NO: 14438 - RNA, 2418 nt, Homo sapiens
  source 1..2418: mol_type = other RNA
gctgggattacaggcatgagccaccgcggccagccataactctgtgactcttgttacaaaggccttatattttgctctttgagggtggttttggtttgatgcctgttggttgccatcttttaactagggatgttttatcaaaatgcccagccaaagtgtccaaacaaattataccttaaagtttgaaaatgtctggcacttctaattcaatgcctgttgtgccaggcactgggctgctgaggaactgagtcccgtccctgcaggctagctagagaacacacacacacacacacacacacacacacacagagtggtcttacaagtcagttttatattctacctatatgcaataaaggtattattatgttgaggtgccttgatataaaaatttttcttaaaggagaggatgcctaaaacaggcattacctgaaacctcctctctccagcattggttgtcttctgtcatgactcagggttttcactgagaatgggatggaaatgtggtctaaagatagggccaatgttgggactggatcccctctgggaagtcagaccaggctagggcaggtccttgaagccatcaggaaaagcctctctgggaggcttatttgctttgagaacatatgtcctgcagttttgttcatatggcagtgaagtttcgtgcacacactctagagccaggcagcctgggttcaaagcgcagctctgccaggtcctaactgcatgaatttgggcaagtcgctcaacctctccatgcctgagtttcctcatcattagcagggatgacagggagtgcaggagtgcggtcgactcccagatattggagagcgctgggctagctgcccattctcccggcctccactcctctttgctgtccagccatcacttgctctttgaaggcaaacaaaacagaaaacagtgccaaaagtatgggaagaaagccagcttctcccctggggtgcctgtgatgccatgcccaccctccctgaccacgcagcccctgtggaccctcagggccccaagcccccatttccatcacatgcgtacacccatgtgtgtccatagccgcccatctcagtcaataaggctgctcctgcccacttggaatagtggtgacaaccaggagtggcttatgggaactatcccaatggcctgacagcatgtccgctgcaaaccgctgaggtaggacactgccctcatgtctagctgatcagcaagaggcgcagttgctttcttaggtaacattgctgctgtgtcctggccattgctggggggtggcacttaatctacaccagaattttccctcctgtatcttccaagctgcttggatcttggtgctgaattaggttggactttgtcttgtggggaagggaggactatagaccctcaacgtaagcaatggtcagactattctaagaaaactcgccgaattaaagcatgaggtaaatttagttctgacttctgtccaccccactgccactgtccccttttatcccatgatcccttgcttttcttttcctcctctctccctatctcttgtgtttgacgcatgataggaattcagaaatatatgtttgtggatttgtttattcacgtagcaaaccatttcttgagtgcctaccatgggccaggtagaatgggcggccccgggctgcagtggtttcttcagcccctctccagggtttacactgtgcaagacggtttgtgatgggtcctcccatcgaggaccacactcttctttctctgtgccccttggtcctcagtctctgaccccacttcaaaggcagcattcactcagggaagctcccatacaatgctagtcagagtaaaagtttggacaaattgccaggaagcagcttgtcagtatgcataaacagcctttaaaatattactactctttgacccagaatttcacttctaggaatctgtcctaaggaagtagtcacatgcaaaagatttatgtaccaagatgttcatcaaagtgttgttttataacaggaagtctcagaagctggataaatatccaacctctggaaatggttagatagaatagtatgtagccattagaaaattatgtctatggggtttaaaatgtcatgggaaaacacttctgacataaaagagcatgagaactgtatatttagcataatcttaactatgttttagaatgcacaggaaaaaaatgtacaaacatattcatagtgatgtctctggtggtaggattatgatcagtaagtacttctgtctcttcatattttcctgtatttgataatacatgcatatgttgtttttaaaataagaaaaattttaagtttaaaattggagctgaaaagtgtttttaggtcaggcgaggtggctcacacctgtaatagcaccactttgggaggctgaggcagtcagatcacttgagcccaggag

SEQ ID NO: 14439 - RNA, 2444 nt, Homo sapiens
  source 1..2444: mol_type = other RNA
gctgggattacaggcatgagccaccgcggccagccataactctgtgactcttgttacaaaggccttatattttgctctttgagggtggttttggtttgatgcctgttggttgccatcttttaactagggatgttttatcaaaatgcccagccaaagtgtccaaacaaattataccttaaagtttgaaaatgtctggcacttctaattcaatgcctgttgtgccaggcactgggctgctgaggaactgagtcccgtccctgcaggctagctagagaacacacacacacacacacacacacacacacacagagtggtcttacaagtcagttttatattctacctatatgcaataaaggtattattatgttgaggtgccttgatataaaaatttttcttaaaggagaggatgcctaaaacaggcattacctgaaacctcctctctccagcattggttgtcttctgtcatgactcagggttttcactgagaatgggatggaaatgtggtctaaagatagggccaatgttgggactggatcccctctgggaagtcagaccaggctagggcaggtccttgaagccatcaggaaaagcctctctgggaggcttatttgctttgagaacatatgtcctgcagttttgttcatatggcagtgaagtttcgtgcacacactctagagccaggcagcctgggttcaaagcgcagctctgccaggtcctaactgcatgaatttgggcaagtcgctcaacctctccatgcctgagtttcctcatctgtaagattggagcaatggtaataccattagcagggatgacagggagtgcaggagtgcggtcgactcccagatattggagagcgctgggctagctgcccattctcccggcctccactcctctttgctgtccagccatcacttgctctttgaaggcaaacaaaacagaaaacagtgccaaaagtatgggaagaaagccagcttctcccctggggtgcctgtgatgccatgcccaccctccctgaccacgcagcccctgtggaccctcagggccccaagcccccatttccatcacatgcgtacacccatgtgtgtccatagccgcccatctcagtcaataaggctgctcctgcccacttggaatagtggtgacaaccaggagtggcttatgggaactatcccaatggcctgacagcatgtccgctgcaaaccgctgaggtaggacactgccctcatgtctagctgatcagcaagaggcgcagttgctttcttaggtaacattgctgctgtgtcctggccattgctggggggtggcacttaatctacaccagaattttccctcctgtatcttccaagctgcttggatcttggtgctgaattaggttggactttgtcttgtggggaagggaggactatagaccctcaacgtaagcaatggtcagactattctaagaaaactcgccgaattaaagcatgaggtaaatttagttctgacttctgtccaccccactgccactgtccccttttatcccatgatcccttgcttttcttttcctcctctctccctatctcttgtgtttgacgcatgataggaattcagaaatatatgtttgtggatttgtttattcacgtagcaaaccatttcttgagtgcctaccatgggccaggtagaatgggcggccccgggctgcagtggtttcttcagcccctctccagggtttacactgtgcaagacggtttgtgatgggtcctcccatcgaggaccacactcttctttctctgtgccccttggtcctcagtctctgaccccacttcaaaggcagcattcactcagggaagctcccatacaatgctagtcagagtaaaagtttggacaaattgccaggaagcagcttgtcagtatgcataaacagcctttaaaatattactactctttgacccagaatttcacttctaggaatctgtcctaaggaagtagtcacatgcaaaagatttatgtaccaagatgttcatcaaagtgttgttttataacaggaagtctcagaagctggataaatatccaacctctggaaatggttagatagaatagtatgtagccattagaaaattatgtctatggggtttaaaatgtcatgggaaaacacttctgacataaaagagcatgagaactgtatatttagcataatcttaactatgttttagaatgcacaggaaaaaaatgtacaaacatattcatagtgatgtctctggtggtaggattatgatcagtaagtacttctgtctcttcatattttcctgtatttgataatacatgcatatgttgtttttaaaataagaaaaattttaagtttaaaattggagctgaaaagtgtttttaggtcaggcgaggtggctcacacctgtaatagcaccactttgggaggctgaggcagtcagatcacttgagcccaggag

SEQ ID NO: 14440 - RNA, 2447 nt, Homo sapiens
  source 1..2447: mol_type = other RNA
gctgggattacaggcatgagccaccgcggccagccataactctgtgactcttgttacaaaggccttatattttgctctttgagggtggttttggtttgatgcctgttggttgccatcttttaactagggatgttttatcaaaatgcccagccaaagtgtccaaacaaattataccttaaagtttgaaaatgtctggcacttctaattcaatgcctgttgtgccaggcactgggctgctgaggaactgagtcccgtccctgcaggctagctagagaacacacacacacacacacacacacacacacacagagtggtcttacaagtcagttttatattctacctatatgcaataaaggtattattatgttgaggtgccttgatataaaaatttttcttaaaggagaggatgcctaaaacaggcattacctgaaacctcctctctccagcattggttgtcttctgtcatgactcagggttttcactgagaatgggatggaaatgtggtctaaagatagggccaatgttgggactggatcccctctgggaagtcagaccaggctagggcaggtccttgaagccatcaggaaaagcctctctgggaggcttatttgctttgagaacatatgtcctgcagttttgttcatatggcagtgaagtttcgtgcacacactctagagccaggcagcctgggttcaaagcgcagctctgccaggtcctaactgcatgaatttgggcaagtcgctcaacctctccatgcctgagtttcctcatctgtaagattggagcaatggtaatacctgcattagcagggatgacagggagtgcaggagtgcggtcgactcccagatattggagagcgctgggctagctgcccattctcccggcctccactcctctttgctgtccagccatcacttgctctttgaaggcaaacaaaacagaaaacagtgccaaaagtatgggaagaaagccagcttctcccctggggtgcctgtgatgccatgcccaccctccctgaccacgcagcccctgtggaccctcagggccccaagcccccatttccatcacatgcgtacacccatgtgtgtccatagccgcccatctcagtcaataaggctgctcctgcccacttggaatagtggtgacaaccaggagtggcttatgggaactatcccaatggcctgacagcatgtccgctgcaaaccgctgaggtaggacactgccctcatgtctagctgatcagcaagaggcgcagttgctttcttaggtaacattgctgctgtgtcctggccattgctggggggtggcacttaatctacaccagaattttccctcctgtatcttccaagctgcttggatcttggtgctgaattaggttggactttgtcttgtggggaagggaggactatagaccctcaacgtaagcaatggtcagactattctaagaaaactcgccgaattaaagcatgaggtaaatttagttctgacttctgtccaccccactgccactgtccccttttatcccatgatcccttgcttttcttttcctcctctctccctatctcttgtgtttgacgcatgataggaattcagaaatatatgtttgtggatttgtttattcacgtagcaaaccatttcttgagtgcctaccatgggccaggtagaatgggcggccccgggctgcagtggtttcttcagcccctctccagggtttacactgtgcaagacggtttgtgatgggtcctcccatcgaggaccacactcttctttctctgtgccccttggtcctcagtctctgaccccacttcaaaggcagcattcactcagggaagctcccatacaatgctagtcagagtaaaagtttggacaaattgccaggaagcagcttgtcagtatgcataaacagcctttaaaatattactactctttgacccagaatttcacttctaggaatctgtcctaaggaagtagtcacatgcaaaagatttatgtaccaagatgttcatcaaagtgttgttttataacaggaagtctcagaagctggataaatatccaacctctggaaatggttagatagaatagtatgtagccattagaaaattatgtctatggggtttaaaatgtcatgggaaaacacttctgacataaaagagcatgagaactgtatatttagcataatcttaactatgttttagaatgcacaggaaaaaaatgtacaaacatattcatagtgatgtctctggtggtaggattatgatcagtaagtacttctgtctcttcatattttcctgtatttgataatacatgcatatgttgtttttaaaataagaaaaattttaagtttaaaattggagctgaaaagtgtttttaggtcaggcgaggtggctcacacctgtaatagcaccactttgggaggctgaggcagtcagatcacttgagcccaggag

SEQ ID NO: 14441 - RNA, 3512 nt, Homo sapiens
  source 1..3512: mol_type = other RNA
gctgggattacaggcatgagccaccgcggccagccataactctgtgactcttgttacaaaggccttatattttgctctttgagggtggttttggtttgatgcctgttggttgccatcttttaactagggatgttttatcaaaatgcccagccaaagtgtccaaacaaattataccttaaagtttgaaaatgtctggcacttctaattcaatgcctgttgtgccaggcactgggctgctgaggaactgagtcccgtccctgcaggctagctagagaacacacacacacacacacacacacacacacacagagtggtcttacaagtcagttttatattctacctatatgcaataaaggtattattatgttgaggtgccttgatataaaaatttttcttaaaggagaggatgcctaaaacaggcattacctgaaacctcctctctccagcattggttgtcttctgtcatgactcagggttttcactgagaatgggatggaaatgtggtctaaagatagggccaatgttgggactggatcccctctgggaagtcagaccaggctagggcaggtccttgaagccatcaggaaaagcctctctgggaggcttatttgctttgagaacatatgtcctgcagttttgttcatatggcagtgaagtttcgtgcacacactctagagccaggcagcctgggttcaaagcgcagctctgccaggtcctaactgcatgaatttgggcaagtcgctcaacctctccatgcctgagtttcctcatctgtaagattggagcaatggtaatacctgctttttagggttgagaagagaattaaatgaattaagatgggtaaagtgcttagagtggagctttgcaagtagtaagtgctatgtaagtgttcgatttaaaatgaaagacccttaaatacattctttgttcatttcacaagcccttcatttcacaaccttacatttcacaaccaagctctgtctcccctggaatccagccataactctgctcacaagtgtgagacaggccccagcagagctgcacgaagaggagagaaggcagccccccagactcccaaccccctgtccaagatggcaaaaccagaacacagcctctgtaccaccccagcaggtattcagaatctgcaatctccaaagcccacttcaattgtaaatgtagagccacgtgcgctttaagtcacctgtcactctggaggctcttttgctcagttcctcaccattagcagggatgacagggagtgcaggagtgcggtcgactcccagatattggagagcgctgggctagctgcccattctcccggcctccactcctctttgctgtccagccatcacttgctcttccccaccccctcggaactcagaggtggtgcaggaatttggactccaagaattaacagctccaccaccatcaccagagccaaaactcaggatgcatgtgcttcatctgctgcttatttccagctgagagccagtggtgccatggttccttagggagccggtcccctgatgccggctcctggccccaaatctctctgatccgggctcttccagaatgtcttgtctccaccatcgcctttgaccaatggtgtccctttgcctggtaatgtcccctttgcctgatgatggccctgtcactcctctctttagcacagaggaggctgtttcatcccttcaagcctgccctcccttcaagtcttagctcaagttcaccttctccgcagagccttctccaatcttcttgactacgtctcctctcagctccagcaacctctgtctctggcactgattccttacttagctaagagaatcacagacacttggggctcaggacaatctgctttctctcttcttacccatggccttggactgtgtgtacctctttgtctccactcccaaacccaacccccagagggcagagagcatgttgtctgtccctttgctcagcatgaagccatgcgtgtggtagatcggcagagttccataacttgtgttgaccgaggggtcactttgctctgaaattacccctgtgtccttcagtatttgcacagatagcttcctggccagaccgaatatatccaagggcatggcccacctctgctcctgtttccaggtccctggtgggggttagttcatgccttcctcataatctgcccactggcctggtcctcaaggtcttcccaactgctcagccagagttgagaaaatgggtcgctccatcctgtttgtgtcgttctctccttcctggcccactctcctgcccacaggtatccaggggctgcctgtagcattagaggacatacatgcacatgcgtgggcatgggacactcacgtagcctccaagcacagcatcaataatgcattctgtgctttatagcatggaaagctgctctaaactttattacacagtggacatgtctgaagcagctcccaaatccacccctgagtgtgttggaattggcaagcctatcacttgggagtctagtttttttgttcgttaataatagatgcttcctgtggccccagcttggcaattttgatttaaagtgatcttaactgaagagactaatggacgggtctgaatttgtgccttttaagcacaaagtattgctcttaattaactggattctatcctttgagcaggcagaggccttcccccaagggcgtcattaacgatccacatctggacatcttccaaagccttcttctgtttcaggccaaccgcaggtgtgttcctgaacacccaggaggctatgagagccacatatgcctcccaaatacacacagtgtgcatgcccagggacatagagcagtgtgcaaagtcccattccatctctctccacctgggagaggatggctcttctgtctgattcatggctcaaagtggtaaaggagctccccactccccgtcccacgcctactcagagtctgcaaatatgtatgcgatatgagagctcgtcagttagctgtcttcagtgtggcgcacatttgaggagtctgactcccctccagcacaggccaatgtgcactgctctcctatctttgtacccccactgttgcactgtgcagaggttggagccatagaagtaccagagctgtgaaaggagaggccccctctcacctctgccctggtctccatccccactttctctaggaagctagtaggtgctgacaggggagagaagggaggggaggggtccagaaacagtggctcatgcctgcaatcctagcactttgggaggctgaggcaggaggatcatttgaggtcaggagtttgagaccagcctgggcaatgtagcaagaccctatctctacaaaaagaaaaaatgtaattagctgggtgtggtggtgggcacctgtagtcctagctacttgggaggatgaggtgggaggattgcttgagcccaagagtttgaggttacagtaagctgtgattgcaccactgcactccagcctgggcaacagagctgagaccctatctcaaaaaaagaaaaa

SEQ ID NO: 14442 - RNA, 2480 nt, Homo sapiens
  source 1..2480: mol_type = other RNA
gctgggattacaggcatgagccaccgcggccagccataactctgtgactcttgttacaaaggccttatattttgctctttgagggtggttttggtttgatgcctgttggttgccatcttttaactagggatgttttatcaaaatgcccagccaaagtgtccaaacaaattataccttaaagtttgaaaatgtctggcacttctaattcaatgcctgttgtgccaggcactgggctgctgaggaactgagtcccgtccctgcaggctagctagagaacacacacacacacacacacacacacacacacagagtggtcttacaagtcagttttatattctacctatatgcaataaaggtattattatgttgaggtgccttgatataaaaatttttcttaaaggagaggatgcctaaaacaggcattacctgaaacctcctctctccagcattggttgtcttctgtcatgactcagggttttcactgagaatgggatggaaatgtggtctaaagatagggccaatgttgggactggatcccctctgggaagtcagaccaggctagggcaggtccttgaagccatcaggaaaagcctctctgggaggcttatttgctttgagaacatatgtcctgcagttttgttcatatggcagtgaagtttcgtgcacacactctagagccaggcagcctgggttcaaagcgcagctctgccaggtcctaactgcatgaatttgggcaagtcgctcaacctctccatgcctgagtttcctcatctgtaagattggagcaatggtaatacctgtcactctggaggctcttttgctcagttcctcaccattagcagggatgacagggagtgcaggagtgcggtcgactcccagatattggagagcgctgggctagctgcccattctcccggcctccactcctctttgctgtccagccatcacttgctctttgaaggcaaacaaaacagaaaacagtgccaaaagtatgggaagaaagccagcttctcccctggggtgcctgtgatgccatgcccaccctccctgaccacgcagcccctgtggaccctcagggccccaagcccccatttccatcacatgcgtacacccatgtgtgtccatagccgcccatctcagtcaataaggctgctcctgcccacttggaatagtggtgacaaccaggagtggcttatgggaactatcccaatggcctgacagcatgtccgctgcaaaccgctgaggtaggacactgccctcatgtctagctgatcagcaagaggcgcagttgctttcttaggtaacattgctgctgtgtcctggccattgctggggggtggcacttaatctacaccagaattttccctcctgtatcttccaagctgcttggatcttggtgctgaattaggttggactttgtcttgtggggaagggaggactatagaccctcaacgtaagcaatggtcagactattctaagaaaactcgccgaattaaagcatgaggtaaatttagttctgacttctgtccaccccactgccactgtccccttttatcccatgatcccttgcttttcttttcctcctctctccctatctcttgtgtttgacgcatgataggaattcagaaatatatgtttgtggatttgtttattcacgtagcaaaccatttcttgagtgcctaccatgggccaggtagaatgggcggccccgggctgcagtggtttcttcagcccctctccagggtttacactgtgcaagacggtttgtgatgggtcctcccatcgaggaccacactcttctttctctgtgccccttggtcctcagtctctgaccccacttcaaaggcagcattcactcagggaagctcccatacaatgctagtcagagtaaaagtttggacaaattgccaggaagcagcttgtcagtatgcataaacagcctttaaaatattactactctttgacccagaatttcacttctaggaatctgtcctaaggaagtagtcacatgcaaaagatttatgtaccaagatgttcatcaaagtgttgttttataacaggaagtctcagaagctggataaatatccaacctctggaaatggttagatagaatagtatgtagccattagaaaattatgtctatggggtttaaaatgtcatgggaaaacacttctgacataaaagagcatgagaactgtatatttagcataatcttaactatgttttagaatgcacaggaaaaaaatgtacaaacatattcatagtgatgtctctggtggtaggattatgatcagtaagtacttctgtctcttcatattttcctgtatttgataatacatgcatatgttgtttttaaaataagaaaaattttaagtttaaaattggagctgaaaagtgtttttaggtcaggcgaggtggctcacacctgtaatagcaccactttgggaggctgaggcagtcagatcacttgagcccaggag

SEQ ID NO: 14443 - RNA, 2454 nt, Homo sapiens
  source 1..2454: mol_type = other RNA
gctgggattacaggcatgagccaccgcggccagccataactctgtgactcttgttacaaaggccttatattttgctctttgagggtggttttggtttgatgcctgttggttgccatcttttaactagggatgttttatcaaaatgcccagccaaagtgtccaaacaaattataccttaaagtttgaaaatgtctggcacttctaattcaatgcctgttgtgccaggcactgggctgctgaggaactgagtcccgtccctgcaggctagctagagaacacacacacacacacacacacacacacacacagagtggtcttacaagtcagttttatattctacctatatgcaataaaggtattattatgttgaggtgccttgatataaaaatttttcttaaaggagaggatgcctaaaacaggcattacctgaaacctcctctctccagcattggttgtcttctgtcatgactcagggttttcactgagaatgggatggaaatgtggtctaaagatagggccaatgttgggactggatcccctctgggaagtcagaccaggctagggcaggtccttgaagccatcaggaaaagcctctctgggaggcttatttgctttgagaacatatgtcctgcagttttgttcatatggcagtgaagtttcgtgcacacactctagagccaggcagcctgggttcaaagcgcagctctgccaggtcctaactgcatgaatttgggcaagtcgctcaacctctccatgcctgagtttcctcatctgtcactctggaggctcttttgctcagttcctcaccattagcagggatgacagggagtgcaggagtgcggtcgactcccagatattggagagcgctgggctagctgcccattctcccggcctccactcctctttgctgtccagccatcacttgctctttgaaggcaaacaaaacagaaaacagtgccaaaagtatgggaagaaagccagcttctcccctggggtgcctgtgatgccatgcccaccctccctgaccacgcagcccctgtggaccctcagggccccaagcccccatttccatcacatgcgtacacccatgtgtgtccatagccgcccatctcagtcaataaggctgctcctgcccacttggaatagtggtgacaaccaggagtggcttatgggaactatcccaatggcctgacagcatgtccgctgcaaaccgctgaggtaggacactgccctcatgtctagctgatcagcaagaggcgcagttgctttcttaggtaacattgctgctgtgtcctggccattgctggggggtggcacttaatctacaccagaattttccctcctgtatcttccaagctgcttggatcttggtgctgaattaggttggactttgtcttgtggggaagggaggactatagaccctcaacgtaagcaatggtcagactattctaagaaaactcgccgaattaaagcatgaggtaaatttagttctgacttctgtccaccccactgccactgtccccttttatcccatgatcccttgcttttcttttcctcctctctccctatctcttgtgtttgacgcatgataggaattcagaaatatatgtttgtggatttgtttattcacgtagcaaaccatttcttgagtgcctaccatgggccaggtagaatgggcggccccgggctgcagtggtttcttcagcccctctccagggtttacactgtgcaagacggtttgtgatgggtcctcccatcgaggaccacactcttctttctctgtgccccttggtcctcagtctctgaccccacttcaaaggcagcattcactcagggaagctcccatacaatgctagtcagagtaaaagtttggacaaattgccaggaagcagcttgtcagtatgcataaacagcctttaaaatattactactctttgacccagaatttcacttctaggaatctgtcctaaggaagtagtcacatgcaaaagatttatgtaccaagatgttcatcaaagtgttgttttataacaggaagtctcagaagctggataaatatccaacctctggaaatggttagatagaatagtatgtagccattagaaaattatgtctatggggtttaaaatgtcatgggaaaacacttctgacataaaagagcatgagaactgtatatttagcataatcttaactatgttttagaatgcacaggaaaaaaatgtacaaacatattcatagtgatgtctctggtggtaggattatgatcagtaagtacttctgtctcttcatattttcctgtatttgataatacatgcatatgttgtttttaaaataagaaaaattttaagtttaaaattggagctgaaaagtgtttttaggtcaggcgaggtggctcacacctgtaatagcaccactttgggaggctgaggcagtcagatcacttgagcccaggag

SEQ ID NO: 14444 - RNA, 1105 nt, Homo sapiens
  source 1..1105: mol_type = other RNA
gctgggattacaggcatgagccaccgcggccagccataactctgtgactcttgttacaaaggccttatattttgctctttgagggtggttttggtttgatgcctgttggttgccatcttttaactagggatgttttatcaaaatgcccagccaaagtgtccaaacaaattataccttaaagtttgaaaatgtctggcacttctaattgaatgcctattgtgccaggcactgggctgctgaggaactgagtcccgtccctgcaggctagctagagaacacacacacacacacacagagtggtcttacaagtcagttttatattctacctatatgcaataaaggtattattatgttgaggtgccttgatataaaaatttttcttaaaggagaggatgcctaaaacaggcattacctgaaacctcctctctccagcattggttgtcttctgtcatgactcagggttttcactgagaatgggatggaaatgtggtctaaagatagggccaatgttgggactggatcccctctgggaagtcagaccaggctagggcaggtccttgaagccatcaggaaaagcctctctgggaggcttatttgctttgagaacatatgtcctgcagttttgttcatatggcagtgaagtttcgtgcacacactctagagccaggcagcctgggttcaaagcgcagctctgccaggtcctaactgcatgaatttgggcaagtcactcaacctctccatgcctgagtttcctcatctgtaagattggagcaatggtaataccattagcagggatgacagggagtgcaggagtgcggtcgactcccagatattggagagcgctgggctagctgcccattctcccggcctccactcctctttgctgtccagccatcacttgctctttgaaggcaaacaaaacagaaaacagtgccaaaagtatgggaagaaagccagcttctcccctggggtgcctgtgatgccatgcccaccctccctgaccacgcagcccctggggaccctcagggccccaagcccccatttccatcacatgcgtacacccatgtgtgtccatagccgcccatctcagtcaataaggctgctc

SEQ ID NO: 14445 - RNA, 1108 nt, Homo sapiens
  source 1..1108: mol_type = other RNA
gctgggattacaggcatgagccaccgcggccagccataactctgtgactcttgttacaaaggccttatattttgctctttgagggtggttttggtttgatgcctgttggttgccatcttttaactagggatgttttatcaaaatgcccagccaaagtgtccaaacaaattataccttaaagtttgaaaatgtctggcacttctaattgaatgcctattgtgccaggcactgggctgctgaggaactgagtcccgtccctgcaggctagctagagaacacacacacacacacacagagtggtcttacaagtcagttttatattctacctatatgcaataaaggtattattatgttgaggtgccttgatataaaaatttttcttaaaggagaggatgcctaaaacaggcattacctgaaacctcctctctccagcattggttgtcttctgtcatgactcagggttttcactgagaatgggatggaaatgtggtctaaagatagggccaatgttgggactggatcccctctgggaagtcagaccaggctagggcaggtccttgaagccatcaggaaaagcctctctgggaggcttatttgctttgagaacatatgtcctgcagttttgttcatatggcagtgaagtttcgtgcacacactctagagccaggcagcctgggttcaaagcgcagctctgccaggtcctaactgcatgaatttgggcaagtcactcaacctctccatgcctgagtttcctcatctgtaagattggagcaatggtaatacctgcattagcagggatgacagggagtgcaggagtgcggtcgactcccagatattggagagcgctgggctagctgcccattctcccggcctccactcctctttgctgtccagccatcacttgctctttgaaggcaaacaaaacagaaaacagtgccaaaagtatgggaagaaagccagcttctcccctggggtgcctgtgatgccatgcccaccctccctgaccacgcagcccctggggaccctcagggccccaagcccccatttccatcacatgcgtacacccatgtgtgtccatagccgcccatctcagtcaataaggctgctc

SEQ ID NO: 14446 - RNA, 2773 nt, Homo sapiens
  source 1..2773: mol_type = other RNA
gctgggattacaggcatgagccaccgcggccagccataactctgtgactcttgttacaaaggccttatattttgctctttgagggtggttttggtttgatgcctgttggttgccatcttttaactagggatgttttatcaaaatgcccagccaaagtgtccaaacaaattataccttaaagtttgaaaatgtctggcacttctaattgaatgcctattgtgccaggcactgggctgctgaggaactgagtcccgtccctgcaggctagctagagaacacacacacacacacacagagtggtcttacaagtcagttttatattctacctatatgcaataaaggtattattatgttgaggtgccttgatataaaaatttttcttaaaggagaggatgcctaaaacaggcattacctgaaacctcctctctccagcattggttgtcttctgtcatgactcagggttttcactgagaatgggatggaaatgtggtctaaagatagggccaatgttgggactggatcccctctgggaagtcagaccaggctagggcaggtccttgaagccatcaggaaaagcctctctgggaggcttatttgctttgagaacatatgtcctgcagttttgttcatatggcagtgaagtttcgtgcacacactctagagccaggcagcctgggttcaaagcgcagctctgccaggtcctaactgcatgaatttgggcaagtcactcaacctctccatgcctgagtttcctcatctgtaagattggagcaatggtaatacctgctttttagggttgagaagagaattaaatgaattaagatgggtaaagtgcttagagtggagctttgcaagtagtaagtgctatgtaagtgtttgatttaaaatgaaagacccttaaatacattctttgttcatttcacaagcccttcatttcacaaccttacatttcacaaccaagctctgtctcccctggaatccagccataactctgctcacaagtgtgagacaggccccagcagagctgcacgaagaggagagaaggcagcccccccagactcccaaccccctgtccaagatggcaaaaccagaacacagcctctgtaccaccccagcaggtgttcagaatctgcaatctccaaagcccacttcaattgtaagtgtagagccacgtgcgctttaagtcacctgtcactctggaggctcttttgctcagttcctcaccattagcagggatgacagggagtgcaggagtgcggtcgactcccagatattggagagcgctgggctagctgcccattctcccggcctccactcctctttgctgtccagccatcacttgctcttccccaccccctcggaactcagaggtggtgcaggaatttggactccaagaattaacagctccaccaccatcaccagagccaaaactcaggatgcatgcgcttcatctgctgcttatttccagctgagagccagtggtgccatggttccttagggagccggtcccctgatgctggctcctggccccaaatctctctgatccgggctcctccagaatgtcttgtctccaccatcgcctttgaccaatggtgtccctttgcctggtaatgtcccctttgcctgatgattgccctgtcactcctctctttagcacagaggaggctgtttcatcccttcaagcctgccctcccttcaagtcttagctcaagttcactttctccgcagagccttctccaatcttcttgactacgtctcctctcagctccagcaacctctgtctctggcactgattccttacttagctaagagaatcacagacacttggggctcaggacaatctgctttctctcttcttacccatggccttggaccgtgtgtacctctttgtctccactcccaaacccaacccccagagggcagagagcatgttgtctgtccctttgctcagcatgaagccatgcgtgtggtagatcggcagagttccataacttgtgttgaccaaggggtcgctttgctctgaaattacccctgtgtccttcagtatttgcacagatagcttcctggccagaccgaatatatccaagggcatggcccacctctgctcctgtttccaggtccctggtgggggttagttcatgccttcctcataatctgcccactggcctggtcctcaaggtcttcccaactgctcagccagagttgagaaaatgggtcgctccatcctgtttgtgtcgttctctccttcctggcccactctcctgcccacaggtatccaggggctgcctgtagcattagaggacatacatgcacatgcgtgggcatgggacactcacgtagcctccaagcacagcatcaataatgcattctgtgctttatagcatggaaagctgctctaaactttattacacagtggacatgtctgaagcagctcccaaatccacccctgagtgtgttggaattggcgagcctatcacttgggagtctagttttctctgttcgttaataatagatgcttcctgtggccccagcttggcaattttgatttaaagtgatcttaactgaagagactaatggacgggtctgaatttgtgccttttaagcacaaagtattgctcttaattaactggattctatcctttgagcaggcagaggccttcccccaatggcgtcattaacgatccacatctggacatcttccaaagccttcttctgtttcaggccaaccgcaggtgtgttcctgaacacccaggaggctatgagagccacatat

SEQ ID NO: 14447 - RNA, 2138 nt, Homo sapiens
  source 1..2138: mol_type = other RNA
gctgggattacaggcatgagccaccgcggccggcaggtctttcctacattttttatttccgtaaggagtctctgcagtgtgagttcttgtatgaaccatgaatttgagaccacgctgaaggctttgtcatattccttttagattcgcagtttctctccagggtgagaacaaatgtctactcaagatgaatgaagatgaaaggctttctgtagactttaccttcacagggttttttttcacatttctgtaagatacgagagttcagggaagatgttctcactcatgctaaccccttgagctcccttccaatatgtcctcctcacatgtttggtacagtcagaaaattaatgaaaaattttccaccttcctttcattcacagggcttctcatctttgtgagtcttaagatgttttttaagtcctgacgactttgcaaagtcttttccacatgtcttacatttatagggtttctctccagtgtggctccttatatgtgtatattttgaggactcccgaatgactttcccacattcttcacattcgtagggcttcttctgcacaacatgctttcttaaatgtttattaaggtgtaaggaatatctaaaggctttcccacatttcccacattcatacggtttctctccagtgtgaattttcatatgtctcataaggaatgactgataaaaaaaggctctcccacattcggggcatttatgggttttctctccagtgcaatgactcttgtgtgaaccggaatttggagcgttggcagaggttgccccagtttgacaatccttcttgtttgtctctgcggtatacaactgcatctgcatggcgtgaattgagttatttctggaggtgttctcgcactgagtaaaatcatacattttctctcgaccatgagtgttgtgtgccctaagggatccgtcttcacggaaagcttttccaaatggattccgctggtgcctgttggcccccgtatcaatttcatcacgtatatgatgcacagtgttctgactgccagtccatgtgcttgatttcagctctgtttttctcccacacggaacccactgaatgttccaccccaagactccatcgtcttcgttgttttcatgtgttttttgactatcgtttaagacaggattatacttgaaaatacttgagtcacgtgttaggatacattgtcttatggaatctccctgtgaaggcacaagcctgcaggtaggtttagagtggttcctcatttcatgatcttcacaaatgctaacaggagattcatctttctcaggggcaactgcaggtggcttcacattattcaccccctgcctgtgtggttcctctgttttggggcatctccagtcttctcttaatgtggagtgctgggaactgatgctcgtgagacacactctgttggcttcaggaaatgttcttttaggaagaatatccggctgaggggttgcgtctttggttttacatggagttgcccaatctatgaatgccaagttcctagaattttccagcatcacgtctctgtagagattcctctgagctgggtccagcagggtccactcctctttggtgaagttcacagccacgtctgcgaaggtcaccgagtcccgtgagtgtgggcgggtgcctgtagtctcagctacccgggaggctgaggagggaggattgcctgagcctgggaggtggaggttgcaataagctatgatcctcccactgcagtccagcctgggcaacagagcaagaccctgggacatatttgtcaccaacgtgacggccagtcctggcttccccgtgtttccttcaaggaggcaggtgaggcagagtcttccactagctccggcttccagatgtctctgtcggtggcgcagcccaaaagcgcgcgcagcccaggagcgtctcggagctgcaccaggatggggatcaaatccccaggcactcctgatccaagcaggaaaccccagccttgggtcctcgctgtcgcctccgcccgcgccaccgttcctaggctctccagctgggaagcgcgctctctgcgcagccaacgcgcctccttgcgggctccggagactccggccgcttgctggcttcctgcatttcccaaggaaagaaggcttttttttcccctcagta

SEQ ID NO: 14448 - RNA, 2009 nt, Homo sapiens
  source 1..2009: mol_type = other RNA
gctgggattacaggcatgagccaccgcggccggcaggtctttcctacattttttatttccgtaaggagtctctgcagtgtgagttcttgtatgaaccatgaatttgagaccacgctgaaggctttgtcatattccttttagattcgcagtttctctccagggtgagaacaaatgtctactcaagatgaatgaagatgaaaggctttctgtagactttaccttcacagggttttttttcacatttctgtaagatacgagagttcagggaagatgttctcactcatgctaaccccttgagctcccttccaatatgtcctcctcacatgtttggtacagtcagaaaattaatgaaaaattttccaccttcctttcattcacagggcttctcatctttgtgagtcttaagatgttttttaagtcctgacgactttgcaaagtcttttccacatgtcttacatttatagggtttctctccagtgtggctccttatatgtgtatattttgaggactcccgaatgactttcccacattcttcacattcgtagggcttcttctgcacaacatgctttcttaaatgtttattaaggtgtaaggaatatctaaaggctttcccacatttcccacattcatacggtttctctccagtgtgaattttcatatgtctcataaggaatgactgataaaaaaaggctctcccacattcggggcatttatgggttttctctccagtgcaatgactcttgtgtgaaccggaatttggagcgttggcagaggttgccccagtttgacaatccttcttgtttgtctctgcggtatacaactgcatctgcatggcgtgaattgagttatttctggaggtgttctcgcactgagtaaaatcatacattttctctcgaccatgagtgttgtgtgccctaagggatccgtcttcacggaaagcttttccaaatggattccgctggtgcctgttggcccccgtatcaatttcatcacgtatatgatgcacagtgttctgactgccagtccatgtgcttgatttcagctctgtttttctcccacacggaacccactgaatgttccaccccaagactccatcgtcttcgttgttttcatgtgttttttgactatcgtttaagacaggattatacttgaaaatacttgagtcacgtgttaggatacattgtcttatggaatctccctgtgaaggcacaagcctgcaggtaggtttagagtggttcctcatttcatgatcttcacaaatgctaacaggagattcatctttctcaggggcaactgcaggtggcttcacattattcaccccctgcctgtgtggttcctctgttttggggcatctccagtcttctcttaatgtggagtgctgggaactgatgctcgtgagacacactctgttggcttcaggaaatgttcttttaggaagaatatccggctgaggggttgcgtctttggttttacatggagttgcccaatctatgaatgccaagttcctagaattttccagcatcacgtctctgtagagattcctctgagctgggtccagcagggtccactcctctttggtgaagttcacagccacgtctgcgaaggtcaccgagtcccgtgagtgtgggcgggtgcctgtagtctcagctacccgggaggctgaggagggaggattgcctgagcctgggaggtggaggttgcaataagctatgatcctcccactgcagtccagcctgggcaacagagcaagaccctgggacatatttgtcaccaacgtgacggccagtcctggcttccccgtgtttccttcaaggaggcaggtgaggcagagtcttccactagctccggcttccagatgtctctgtcggtggcgcagcccaaaagcgcgcgcagcccaggagcgtctcggagtccccaggcactcctgatccaagcaggaaaccccagccttgggtcctcgctgtcgcctccgcccgcgccaccgttcctaggctctccagctgggaagc

SEQ ID NO: 14449 - RNA, 2034 nt, Homo sapiens
  source 1..2034: mol_type = other RNA
gctgggattacaggcatgagccaccgcggccggcaggtctttcctacattttttatttccgtaaggagtctctgcagtgtgagttcttgtatgaaccatgaatttgagaccacgctgaaggctttgtcatattccttttagattcgcagtttctctccagggtgagaacaaatgtctactcaagatgaatgaagatgaaaggctttctgtagactttaccttcacagggttttttttcacatttctgtaagatacgagagttcagggaagatgttctcactcatgctaaccccttgagctcccttccaatatgtcctcctcacatgtttggtacagtcagaaaattaatgaaaaattttccaccttcctttcattcacagggcttctcatctttgtgagtcttaagatgttttttaagtcctgacgactttgcaaagtcttttccacatgtcttacatttatagggtttctctccagtgtggctccttatatgtgtatattttgaggactcccgaatgactttcccacattcttcacattcgtagggcttcttctgcacaacatgctttcttaaatgtttattaaggtgtaaggaatatctaaaggctttcccacatttcccacattcatacggtttctctccagtgtgaattttcatatgtctcataaggaatgactgataaaaaaaggctctcccacattcggggcatttatgggttttctctccagtgcaatgactcttgtgtgaaccggaatttggagcgttggcagaggttgccccagtttgacaatccttcttgtttgtctctgcggtatacaactgcatctgcatggcgtgaattgagttatttctggaggtgttctcgcactgagtaaaatcatacattttctctcgaccatgagtgttgtgtgccctaagggatccgtcttcacggaaagcttttccaaatggattccgctggtgcctgttggcccccgtatcaatttcatcacgtatatgatgcacagtgttctgactgccagtccatgtgcttgatttcagctctgtttttctcccacacggaacccactgaatgttccaccccaagactccatcgtcttcgttgttttcatgtgttttttgactatcgtttaagacaggattatacttgaaaatacttgagtcacgtgttaggatacattgtcttatggaatctccctgtgaaggcacaagcctgcaggtaggtttagagtggttcctcatttcatgatcttcacaaatgctaacaggagattcatctttctcaggggcaactgcaggtggcttcacattattcaccccctgcctgtgtggttcctctgttttggggcatctccagtcttctcttaatgtggagtgctgggaactgatgctcgtgagacacactctgttggcttcaggaaatgttcttttaggaagaatatccggctgaggggttgcgtctttggttttacatggagttgcccaatctatgaatgccaagttcctagaattttccagcatcacgtctctgtagagattcctctgagctgggtccagcagggtccactcctctttggtgaagttcacagccacgtctgcgaaggtcaccgagtcctgggacatatttgtcaccaacgtgacggccagtcctggcttccccgtgtttccttcaaggaggcaggtgaggcagagctgtaatcccagctactagagaggttgaggcaggagaattacttgaacctggaaggcagaggttgcggtgagacgagattgcaccactgcactccagctcttccactagctccggcttccagatgtctctgtcggtggcgcagcccaaaagcgcgcgcagcccaggagcgtctcggagtccccaggcactcctgatccaagcaggaaaccccagccttgggtcctcgctgtcgcctccgcccgcgccaccgttcctaggctctccagctgggaagcgcgctctctgcgcagccaacgcgcctccttgcgggctccggagactccggccgcttgctggcttc

SEQ ID NO: 14450 - RNA, 2139 nt, Homo sapiens
  source 1..2139: mol_type = other RNA
gctgggattacaggcatgagccaccgcggccggcaggtctttcctacattttttatttccgtaaggagtctctgcagtgtgagttcttgtatgaaccatgaatttgagaccacgctgaaggctttgtcatattccttttagattcgcagtttctctccagggtgagaacaaatgtctactcaagatgaatgaagatgaaaggctttctgtagactttaccttcacagggttttttttcacatttctgtaagatacgagagttcagggaagatgttctcactcatgctaaccccttgagctcccttccaatatgtcctcctcacatgtttggtacagtcagaaaattaatgaaaaattttccaccttcctttcattcacagggcttctcatctttgtgagtcttaagatgttttttaagtcctgacgactttgcaaagtcttttccacatgtcttacatttatagggtttctctccagtgtggctccttatatgtgtatattttgaggactcccgaatgactttcccacattcttcacattcgtagggcttcttctgcacaacatgctttcttaaatgtttattaaggtgtaaggaatatctaaaggctttcccacatttcccacattcatacggtttctctccagtgtgaattttcatatgtctcataaggaatgactgataaaaaaaggctctcccacattcggggcatttatgggttttctctccagtgcaatgactcttgtgtgaaccggaatttggagcgttggcagaggttgccccagtttgacaatccttcttgtttgtctctgcggtatacaactgcatctgcatggcgtgaattgagttatttctggaggtgttctcgcactgagtaaaatcatacattttctctcgaccatgagtgttgtgtgccctaagggatccgtcttcacggaaagcttttccaaatggattccgctggtgcctgttggcccccgtatcaatttcatcacgtatatgatgcacagtgttctgactgccagtccatgtgcttgatttcagctctgtttttctcccacacggaacccactgaatgttccaccccaagactccatcgtcttcgttgttttcatgtgttttttgactatcgtttaagacaggattatacttgaaaatacttgagtcacgtgttaggatacattgtcttatggaatctccctgtgaaggcacaagcctgcaggtaggtttagagtggttcctcatttcatgatcttcacaaatgctaacaggagattcatctttctcaggggcaactgcaggtggcttcacattattcaccccctgcctgtgtggttcctctgttttggggcatctccagtcttctcttaatgtggagtgctgggaactgatgctcgtgagacacactctgttggcttcaggaaatgttcttttaggaagaatatccggctgaggggttgcgtctttggttttacatggagttgcccaatctatgaatgccaagttcctagaattttccagcatcacgtctctgtagagattcctctgagctgggtccagcagggtccactcctctttggtgaagttcacagccacgtctgcgaaggtcaccgagtcctgggacatatttgtcaccaacgtgacggccagtcctggcttccccgtgtttccttcaaggaggcaggtgaggcagagtcttccactagctccggcttccagatgtctctgtcggtggcgcagcccaaaagcgcgcgcagcccaggagcgtctcggagctgcaccaggatggggatcaaatccccaggcactcctgatccaagcaggaaaccccagccttgggtcctcgctgtcgcctccgcccgcgccaccgttcctaggctctccagctgggaagcgcgctctctgcgcagccaacgcgcctccttgcgggctccggagactccggccgcttgctggcttcctgcatttcccaaggaaagaaggcttttttttcccctcagtatatgctgcccagactcgtctcgaactcctgggtgtcacgcgtgtccgtatagaagaccacctaaacaggctttgtgtaagcaacaaaggctgtttattcacttgggtgcaagtgggctgagttggaaaagagagtcagc

SEQ ID NO: 14451 - RNA, 2097 nt, Homo sapiens
  source 1..2097: mol_type = other RNA
gctgggattacaggcatgagccaccgcggccggcaggtctttcctacattttttatttccgtaaggagtctctgcagtgtgagttcttgtatgaaccatgaatttgagaccacgctgaaggctttgtcatattccttttagattcgcagtttctctccagggtgagaacaaatgtctactcaagatgaatgaagatgaaaggctttctgtagactttaccttcacagggttttttttcacatttctgtaagatacgagagttcagggaagatgttctcactcatgctaaccccttgagctcccttccaatatgtcctcctcacatgtttggtacagtcagaaaattaatgaaaaattttccaccttcctttcattcacagggcttctcatctttgtgagtcttaagatgttttttaagtcctgacgactttgcaaagtcttttccacatgtcttacatttatagggtttctctccagtgtggctccttatatgtgtatattttgaggactcccgaatgactttcccacattcttcacattcgtagggcttcttctgcacaacatgctttcttaaatgtttattaaggtgtaaggaatatctaaaggctttcccacatttcccacattcatacggtttctctccagtgtgaattttcatatgtctcataaggaatgactgataaaaaaaggctctcccacattcggggcatttatgggttttctctccagtgcaatgactcttgtgtgaaccggaatttggagcgttggcagaggttgccccagtttgacaatccttcttgtttgtctctgcggtatacaactgcatctgcatggcgtgaattgagttatttctggaggtgttctcgcactgagtaaaatcatacattttctctcgaccatgagtgttgtgtgccctaagggatccgtcttcacggaaagcttttccaaatggattccgctggtgcctgttggcccccgtatcaatttcatcacgtatatgatgcacagtgttctgactgccagtccatgtgcttgatttcagctctgtttttctcccacacggaacccactgaatgttccaccccaagactccatcgtcttcgttgttttcatgtgttttttgactatcgtttaagacaggattatacttgaaaatacttgagtcacgtgttaggatacattgtcttatggaatctccctgtgaaggcacaagcctgcaggtaggtttagagtggttcctcatttcatgatcttcacaaatgctaacaggagattcatctttctcaggggcaactgcaggtggcttcacattattcaccccctgcctgtgtggttcctctgttttggggcatctccagtcttctcttaatgtggagtgctgggaactgatgctcgtgagacacactctgttggcttcaggaaatgttcttttaggaagaatatccggctgaggggttgcgtctttggttttacatggagttgcccaatctatgaatgccaagttcctagaattttccagcatcacgtctctgtagagattcctctgagctgggtccagcagggtccactcctctttggtgaagttcacagccacgtctgcgaaggtcaccgagtcctgggacatatttgtcaccaacgtgacggccagtcctggcttccccgtgtttccttcaaggaggcaggtgaggcagagtcttccactagctccggcttccagatgtctctgtcggtggcgcagcccaaaagcgcgcgcagcccaggagcgtctcggagctgcaccaggatggggatcaaatccccaggcactcctgatccaagcaggaaaccccagccttgggtcctcgctgtcgcctccgcccgcgccaccgttcctaggctctccagctgggaagcgcgctctctgcgcagccaacgcgcctccttgcgggctccggagactccggccgcttgctggcttctatgctgcccagactcgtctcgaactcctgggtgtcacgcgtgtccgtatagaagaccacctaaacaggctttgtgtaagcaacaaaggctgtttattcacttgggtgcaagtgggctgagttggaaaagagagtcagc
